European Patent Application EP 4 803 615 A1, published September 9, 2026. Title: 一种修饰的细胞及其用途. Applicant: 苏州沙砾生物科技有限公司. Application WO. The sequence listing filed with the application follows.

SEQUENCE LISTING (49637 sequences)

SEQ ID NO: 1 - RNA, 20 nt, synthetic construct
  source 1..20: mol_type = other RNA
gtgaattttgagcgaggtga

SEQ ID NO: 2 - RNA, 20 nt, synthetic construct
  source 1..20: mol_type = other RNA
tttcgggtgaattttgagcg

SEQ ID NO: 3 - RNA, 20 nt, synthetic construct
  source 1..20: mol_type = other RNA
ccgaaaatgcgctgagactt

SEQ ID NO: 4 - RNA, 20 nt, synthetic construct
  source 1..20: mol_type = other RNA
caaagtctcagcgcattttc

SEQ ID NO: 5 - RNA, 20 nt, synthetic construct
  source 1..20: mol_type = other RNA
aatgcgctgagactttggca

SEQ ID NO: 6 - RNA, 20 nt, synthetic construct
  source 1..20: mol_type = other RNA
atgcgctgagactttggcat

SEQ ID NO: 7 - RNA, 20 nt, synthetic construct
  source 1..20: mol_type = other RNA
tgcgctgagactttggcatg

SEQ ID NO: 8 - RNA, 20 nt, synthetic construct
  source 1..20: mol_type = other RNA
agcgcttctgtaacgtcagt

SEQ ID NO: 9 - RNA, 20 nt, synthetic construct
  source 1..20: mol_type = other RNA
aagcgcttctgtaacgtcag

SEQ ID NO: 10 - RNA, 20 nt, synthetic construct
  source 1..20: mol_type = other RNA
atgaatttaaaaactgctcc

SEQ ID NO: 11 - RNA, 20 nt, synthetic construct
  source 1..20: mol_type = other RNA
aatttaaaaactgctccagg

SEQ ID NO: 12 - RNA, 20 nt, synthetic construct
  source 1..20: mol_type = other RNA
taaaaactgctccaggcggc

SEQ ID NO: 13 - RNA, 20 nt, synthetic construct
  source 1..20: mol_type = other RNA
aactgctccaggcggccgga

SEQ ID NO: 14 - RNA, 20 nt, synthetic construct
  source 1..20: mol_type = other RNA
tgctccaggcggccggacgg

SEQ ID NO: 15 - RNA, 20 nt, synthetic construct
  source 1..20: mol_type = other RNA
gctccaggcggccggacggc

SEQ ID NO: 16 - RNA, 20 nt, synthetic construct
  source 1..20: mol_type = other RNA
tgtcccgccgtccggccgcc

SEQ ID NO: 17 - RNA, 20 nt, synthetic construct
  source 1..20: mol_type = other RNA
ggaggcgttgtcccgccgtc

SEQ ID NO: 18 - RNA, 20 nt, synthetic construct
  source 1..20: mol_type = other RNA
cctcctcacttgctcctcta

SEQ ID NO: 19 - RNA, 20 nt, synthetic construct
  source 1..20: mol_type = other RNA
ccgtagaggagcaagtgagg

SEQ ID NO: 20 - RNA, 20 nt, synthetic construct
  source 1..20: mol_type = other RNA
ttgccgtagaggagcaagtg

SEQ ID NO: 21 - RNA, 20 nt, synthetic construct
  source 1..20: mol_type = other RNA
aggaaggggccttgccgtag

SEQ ID NO: 22 - RNA, 20 nt, synthetic construct
  source 1..20: mol_type = other RNA
ggccccttccttctccctgc

SEQ ID NO: 23 - RNA, 20 nt, synthetic construct
  source 1..20: mol_type = other RNA
ttccttctccctgccggctg

SEQ ID NO: 24 - RNA, 20 nt, synthetic construct
  source 1..20: mol_type = other RNA
agccggcagggagaaggaag

SEQ ID NO: 25 - RNA, 20 nt, synthetic construct
  source 1..20: mol_type = other RNA
cagccggcagggagaaggaa

SEQ ID NO: 26 - RNA, 20 nt, synthetic construct
  source 1..20: mol_type = other RNA
cttctccctgccggctgcgg

SEQ ID NO: 27 - RNA, 20 nt, synthetic construct
  source 1..20: mol_type = other RNA
caccgcagccggcagggaga

SEQ ID NO: 28 - RNA, 20 nt, synthetic construct
  source 1..20: mol_type = other RNA
tgccggctgcggtggtgtgt

SEQ ID NO: 29 - RNA, 20 nt, synthetic construct
  source 1..20: mol_type = other RNA
gccggctgcggtggtgtgta

SEQ ID NO: 30 - RNA, 20 nt, synthetic construct
  source 1..20: mol_type = other RNA
acacaccaccgcagccggca

SEQ ID NO: 31 - RNA, 20 nt, synthetic construct
  source 1..20: mol_type = other RNA
tacacaccaccgcagccggc

SEQ ID NO: 32 - RNA, 20 nt, synthetic construct
  source 1..20: mol_type = other RNA
ggctgcggtggtgtgtaggg

SEQ ID NO: 33 - RNA, 20 nt, synthetic construct
  source 1..20: mol_type = other RNA
accctacacaccaccgcagc

SEQ ID NO: 34 - RNA, 20 nt, synthetic construct
  source 1..20: mol_type = other RNA
gattaaggaaactctgtaaa

SEQ ID NO: 35 - RNA, 20 nt, synthetic construct
  source 1..20: mol_type = other RNA
ggattaaggaaactctgtaa

SEQ ID NO: 36 - RNA, 20 nt, synthetic construct
  source 1..20: mol_type = other RNA
aggtcaggctagatggatta

SEQ ID NO: 37 - RNA, 20 nt, synthetic construct
  source 1..20: mol_type = other RNA
atctagcctgacctcacctg

SEQ ID NO: 38 - RNA, 20 nt, synthetic construct
  source 1..20: mol_type = other RNA
tctagcctgacctcacctgc

SEQ ID NO: 39 - RNA, 20 nt, synthetic construct
  source 1..20: mol_type = other RNA
gcaggtgaggtcaggctaga

SEQ ID NO: 40 - RNA, 20 nt, synthetic construct
  source 1..20: mol_type = other RNA
aacatcccgcaggtgaggtc

SEQ ID NO: 41 - RNA, 20 nt, synthetic construct
  source 1..20: mol_type = other RNA
aatggaacatcccgcaggtg

SEQ ID NO: 42 - RNA, 20 nt, synthetic construct
  source 1..20: mol_type = other RNA
cgggaaatggaacatcccgc

SEQ ID NO: 43 - RNA, 20 nt, synthetic construct
  source 1..20: mol_type = other RNA
gtgggaggtggatcgggaaa

SEQ ID NO: 44 - RNA, 20 nt, synthetic construct
  source 1..20: mol_type = other RNA
gggggtgtgggaggtggatc

SEQ ID NO: 45 - RNA, 20 nt, synthetic construct
  source 1..20: mol_type = other RNA
cgggggtgtgggaggtggat

SEQ ID NO: 46 - RNA, 20 nt, synthetic construct
  source 1..20: mol_type = other RNA
tgcagcgggggtgtgggagg

SEQ ID NO: 47 - RNA, 20 nt, synthetic construct
  source 1..20: mol_type = other RNA
aactgcagcgggggtgtggg

SEQ ID NO: 48 - RNA, 20 nt, synthetic construct
  source 1..20: mol_type = other RNA
gacaactgcagcgggggtgt

SEQ ID NO: 49 - RNA, 20 nt, synthetic construct
  source 1..20: mol_type = other RNA
agacaactgcagcgggggtg

SEQ ID NO: 50 - RNA, 20 nt, synthetic construct
  source 1..20: mol_type = other RNA
cgctgcagttgtctagaagc

SEQ ID NO: 51 - RNA, 20 nt, synthetic construct
  source 1..20: mol_type = other RNA
cttctagacaactgcagcgg

SEQ ID NO: 52 - RNA, 20 nt, synthetic construct
  source 1..20: mol_type = other RNA
ctgcagttgtctagaagctg

SEQ ID NO: 53 - RNA, 20 nt, synthetic construct
  source 1..20: mol_type = other RNA
agcttctagacaactgcagc

SEQ ID NO: 54 - RNA, 20 nt, synthetic construct
  source 1..20: mol_type = other RNA
cagcttctagacaactgcag

SEQ ID NO: 55 - RNA, 20 nt, synthetic construct
  source 1..20: mol_type = other RNA
agttgtctagaagctggggc

SEQ ID NO: 56 - RNA, 20 nt, synthetic construct
  source 1..20: mol_type = other RNA
gttgtctagaagctggggct

SEQ ID NO: 57 - RNA, 20 nt, synthetic construct
  source 1..20: mol_type = other RNA
ttgtctagaagctggggctg

SEQ ID NO: 58 - RNA, 20 nt, synthetic construct
  source 1..20: mol_type = other RNA
aagctggggctggggaactg

SEQ ID NO: 59 - RNA, 20 nt, synthetic construct
  source 1..20: mol_type = other RNA
ggggctggggaactgaggcg

SEQ ID NO: 60 - RNA, 20 nt, synthetic construct
  source 1..20: mol_type = other RNA
gggctggggaactgaggcgc

SEQ ID NO: 61 - RNA, 20 nt, synthetic construct
  source 1..20: mol_type = other RNA
ctggggaactgaggcgcggg

SEQ ID NO: 62 - RNA, 20 nt, synthetic construct
  source 1..20: mol_type = other RNA
gaggcgcgggaggagcagac

SEQ ID NO: 63 - RNA, 20 nt, synthetic construct
  source 1..20: mol_type = other RNA
gcgcgggaggagcagacagg

SEQ ID NO: 64 - RNA, 20 nt, synthetic construct
  source 1..20: mol_type = other RNA
cgcgggaggagcagacagga

SEQ ID NO: 65 - RNA, 20 nt, synthetic construct
  source 1..20: mol_type = other RNA
ggaggagcagacaggagggc

SEQ ID NO: 66 - RNA, 20 nt, synthetic construct
  source 1..20: mol_type = other RNA
gaggagcagacaggagggcc

SEQ ID NO: 67 - RNA, 20 nt, synthetic construct
  source 1..20: mol_type = other RNA
aggagcagacaggagggccg

SEQ ID NO: 68 - RNA, 20 nt, synthetic construct
  source 1..20: mol_type = other RNA
gcagacaggagggccggggt

SEQ ID NO: 69 - RNA, 20 nt, synthetic construct
  source 1..20: mol_type = other RNA
cagacaggagggccggggtt

SEQ ID NO: 70 - RNA, 20 nt, synthetic construct
  source 1..20: mol_type = other RNA
agacaggagggccggggttg

SEQ ID NO: 71 - RNA, 20 nt, synthetic construct
  source 1..20: mol_type = other RNA
cgtggctggcgccccaaccc

SEQ ID NO: 72 - RNA, 20 nt, synthetic construct
  source 1..20: mol_type = other RNA
ttggggcgccagccacgcgt

SEQ ID NO: 73 - RNA, 20 nt, synthetic construct
  source 1..20: mol_type = other RNA
tggggcgccagccacgcgtt

SEQ ID NO: 74 - RNA, 20 nt, synthetic construct
  source 1..20: mol_type = other RNA
ctgctctcccaacgcgtggc

SEQ ID NO: 75 - RNA, 20 nt, synthetic construct
  source 1..20: mol_type = other RNA
acgcgttgggagagcagacc

SEQ ID NO: 76 - RNA, 20 nt, synthetic construct
  source 1..20: mol_type = other RNA
cgcgttgggagagcagaccc

SEQ ID NO: 77 - RNA, 20 nt, synthetic construct
  source 1..20: mol_type = other RNA
gggtctgctctcccaacgcg

SEQ ID NO: 78 - RNA, 20 nt, synthetic construct
  source 1..20: mol_type = other RNA
agacccgggtgcagactcag

SEQ ID NO: 79 - RNA, 20 nt, synthetic construct
  source 1..20: mol_type = other RNA
cgggtgcagactcagaggac

SEQ ID NO: 80 - RNA, 20 nt, synthetic construct
  source 1..20: mol_type = other RNA
agtcctctgagtctgcaccc

SEQ ID NO: 81 - RNA, 20 nt, synthetic construct
  source 1..20: mol_type = other RNA
cagtcctctgagtctgcacc

SEQ ID NO: 82 - RNA, 20 nt, synthetic construct
  source 1..20: mol_type = other RNA
gcagactcagaggactggag

SEQ ID NO: 83 - RNA, 20 nt, synthetic construct
  source 1..20: mol_type = other RNA
gactcagaggactggagagg

SEQ ID NO: 84 - RNA, 20 nt, synthetic construct
  source 1..20: mol_type = other RNA
agaggactggagaggcggca

SEQ ID NO: 85 - RNA, 20 nt, synthetic construct
  source 1..20: mol_type = other RNA
tggagaggcggcatggagtt

SEQ ID NO: 86 - RNA, 20 nt, synthetic construct
  source 1..20: mol_type = other RNA
cggcatggagtttggtctcc

SEQ ID NO: 87 - RNA, 20 nt, synthetic construct
  source 1..20: mol_type = other RNA
ggcatggagtttggtctcct

SEQ ID NO: 88 - RNA, 20 nt, synthetic construct
  source 1..20: mol_type = other RNA
atggagtttggtctcctggg

SEQ ID NO: 89 - RNA, 20 nt, synthetic construct
  source 1..20: mol_type = other RNA
gtctcctgggaggtagagtg

SEQ ID NO: 90 - RNA, 20 nt, synthetic construct
  source 1..20: mol_type = other RNA
ggaggtagagtgaggtgctg

SEQ ID NO: 91 - RNA, 20 nt, synthetic construct
  source 1..20: mol_type = other RNA
agcacctcactctacctccc

SEQ ID NO: 92 - RNA, 20 nt, synthetic construct
  source 1..20: mol_type = other RNA
agtgaggtgctgcggactcc

SEQ ID NO: 93 - RNA, 20 nt, synthetic construct
  source 1..20: mol_type = other RNA
gtgaggtgctgcggactcca

SEQ ID NO: 94 - RNA, 20 nt, synthetic construct
  source 1..20: mol_type = other RNA
aggtgctgcggactccaggg

SEQ ID NO: 95 - RNA, 20 nt, synthetic construct
  source 1..20: mol_type = other RNA
ctgcggactccagggaggaa

SEQ ID NO: 96 - RNA, 20 nt, synthetic construct
  source 1..20: mol_type = other RNA
tgcggactccagggaggaaa

SEQ ID NO: 97 - RNA, 20 nt, synthetic construct
  source 1..20: mol_type = other RNA
gactccagggaggaaaggga

SEQ ID NO: 98 - RNA, 20 nt, synthetic construct
  source 1..20: mol_type = other RNA
actccagggaggaaagggat

SEQ ID NO: 99 - RNA, 20 nt, synthetic construct
  source 1..20: mol_type = other RNA
ccagggaggaaagggatggg

SEQ ID NO: 100 - RNA, 20 nt, synthetic construct
  source 1..20: mol_type = other RNA
cagggaggaaagggatgggt

SEQ ID NO: 101 - RNA, 20 nt, synthetic construct
  source 1..20: mol_type = other RNA
agggaggaaagggatgggtg

SEQ ID NO: 102 - RNA, 20 nt, synthetic construct
  source 1..20: mol_type = other RNA
gaggaaagggatgggtgggg

SEQ ID NO: 103 - RNA, 20 nt, synthetic construct
  source 1..20: mol_type = other RNA
gaaagggatgggtggggagg

SEQ ID NO: 104 - RNA, 20 nt, synthetic construct
  source 1..20: mol_type = other RNA
aaagggatgggtggggaggc

SEQ ID NO: 105 - RNA, 20 nt, synthetic construct
  source 1..20: mol_type = other RNA
gggatgggtggggaggcggg

SEQ ID NO: 106 - RNA, 20 nt, synthetic construct
  source 1..20: mol_type = other RNA
ggatgggtggggaggcggga

SEQ ID NO: 107 - RNA, 20 nt, synthetic construct
  source 1..20: mol_type = other RNA
gatgggtggggaggcgggag

SEQ ID NO: 108 - RNA, 20 nt, synthetic construct
  source 1..20: mol_type = other RNA
gggtggggaggcgggagggg

SEQ ID NO: 109 - RNA, 20 nt, synthetic construct
  source 1..20: mol_type = other RNA
tggggaggcgggaggggagg

SEQ ID NO: 110 - RNA, 20 nt, synthetic construct
  source 1..20: mol_type = other RNA
ggggaggcgggaggggagga

SEQ ID NO: 111 - RNA, 20 nt, synthetic construct
  source 1..20: mol_type = other RNA
aggcgggaggggaggaggga

SEQ ID NO: 112 - RNA, 20 nt, synthetic construct
  source 1..20: mol_type = other RNA
ggcgggaggggaggagggac

SEQ ID NO: 113 - RNA, 20 nt, synthetic construct
  source 1..20: mol_type = other RNA
gcgggaggggaggagggacg

SEQ ID NO: 114 - RNA, 20 nt, synthetic construct
  source 1..20: mol_type = other RNA
tattttgcgctcccgcaccg

SEQ ID NO: 115 - RNA, 20 nt, synthetic construct
  source 1..20: mol_type = other RNA
ctgagttcgggccgcggtgc

SEQ ID NO: 116 - RNA, 20 nt, synthetic construct
  source 1..20: mol_type = other RNA
gctgagttcgggccgcggtg

SEQ ID NO: 117 - RNA, 20 nt, synthetic construct
  source 1..20: mol_type = other RNA
gaacagctgagttcgggccg

SEQ ID NO: 118 - RNA, 20 nt, synthetic construct
  source 1..20: mol_type = other RNA
aaggcagaacagctgagttc

SEQ ID NO: 119 - RNA, 20 nt, synthetic construct
  source 1..20: mol_type = other RNA
ctcagctgttctgccttcac

SEQ ID NO: 120 - RNA, 20 nt, synthetic construct
  source 1..20: mol_type = other RNA
tcactggcctcagccagtcg

SEQ ID NO: 121 - RNA, 20 nt, synthetic construct
  source 1..20: mol_type = other RNA
cactggcctcagccagtcga

SEQ ID NO: 122 - RNA, 20 nt, synthetic construct
  source 1..20: mol_type = other RNA
cgactggctgaggccagtga

SEQ ID NO: 123 - RNA, 20 nt, synthetic construct
  source 1..20: mol_type = other RNA
ggagctccctcgactggctg

SEQ ID NO: 124 - RNA, 20 nt, synthetic construct
  source 1..20: mol_type = other RNA
cagtcgagggagctcctacg

SEQ ID NO: 125 - RNA, 20 nt, synthetic construct
  source 1..20: mol_type = other RNA
ctcgtaggagctccctcgac

SEQ ID NO: 126 - RNA, 20 nt, synthetic construct
  source 1..20: mol_type = other RNA
gggctcgcagataacctcgt

SEQ ID NO: 127 - RNA, 20 nt, synthetic construct
  source 1..20: mol_type = other RNA
tctgcgagcccagcaaatct

SEQ ID NO: 128 - RNA, 20 nt, synthetic construct
  source 1..20: mol_type = other RNA
ctgcgagcccagcaaatctt

SEQ ID NO: 129 - RNA, 20 nt, synthetic construct
  source 1..20: mol_type = other RNA
tgcgagcccagcaaatcttg

SEQ ID NO: 130 - RNA, 20 nt, synthetic construct
  source 1..20: mol_type = other RNA
gcgagcccagcaaatcttgg

SEQ ID NO: 131 - RNA, 20 nt, synthetic construct
  source 1..20: mol_type = other RNA
taggacccccaagatttgct

SEQ ID NO: 132 - RNA, 20 nt, synthetic construct
  source 1..20: mol_type = other RNA
ctaggacccccaagatttgc

SEQ ID NO: 133 - RNA, 20 nt, synthetic construct
  source 1..20: mol_type = other RNA
gttgcgcactgcatttggct

SEQ ID NO: 134 - RNA, 20 nt, synthetic construct
  source 1..20: mol_type = other RNA
agaacgttgcgcactgcatt

SEQ ID NO: 135 - RNA, 20 nt, synthetic construct
  source 1..20: mol_type = other RNA
gcgcaacgttctctctcact

SEQ ID NO: 136 - RNA, 20 nt, synthetic construct
  source 1..20: mol_type = other RNA
caacgttctctctcacttgg

SEQ ID NO: 137 - RNA, 20 nt, synthetic construct
  source 1..20: mol_type = other RNA
aaaaaaaacgaggtgaatgg

SEQ ID NO: 138 - RNA, 20 nt, synthetic construct
  source 1..20: mol_type = other RNA
aaaaaaaaaaacgaggtgaa

SEQ ID NO: 139 - RNA, 20 nt, synthetic construct
  source 1..20: mol_type = other RNA
tcgtttttttttttcctaaa

SEQ ID NO: 140 - RNA, 20 nt, synthetic construct
  source 1..20: mol_type = other RNA
ttttaggaaaaaaaaaaacg

SEQ ID NO: 141 - RNA, 20 nt, synthetic construct
  source 1..20: mol_type = other RNA
tcagaaaaaaaaatcctttt

SEQ ID NO: 142 - RNA, 20 nt, synthetic construct
  source 1..20: mol_type = other RNA
tgtgcaaagcaggtaaaata

SEQ ID NO: 143 - RNA, 20 nt, synthetic construct
  source 1..20: mol_type = other RNA
atgtgcaaagcaggtaaaat

SEQ ID NO: 144 - RNA, 20 nt, synthetic construct
  source 1..20: mol_type = other RNA
gcgggaggcatgtgcaaagc

SEQ ID NO: 145 - RNA, 20 nt, synthetic construct
  source 1..20: mol_type = other RNA
acatgcctcccgccctcacc

SEQ ID NO: 146 - RNA, 20 nt, synthetic construct
  source 1..20: mol_type = other RNA
catgcctcccgccctcaccc

SEQ ID NO: 147 - RNA, 20 nt, synthetic construct
  source 1..20: mol_type = other RNA
gcctcccgccctcacccggg

SEQ ID NO: 148 - RNA, 20 nt, synthetic construct
  source 1..20: mol_type = other RNA
tcccgccctcacccgggagg

SEQ ID NO: 149 - RNA, 20 nt, synthetic construct
  source 1..20: mol_type = other RNA
gcctcccgggtgagggcggg

SEQ ID NO: 150 - RNA, 20 nt, synthetic construct
  source 1..20: mol_type = other RNA
gccgcctcccgggtgagggc

SEQ ID NO: 151 - RNA, 20 nt, synthetic construct
  source 1..20: mol_type = other RNA
cgccgcctcccgggtgaggg

SEQ ID NO: 152 - RNA, 20 nt, synthetic construct
  source 1..20: mol_type = other RNA
cttcgccgcctcccgggtga

SEQ ID NO: 153 - RNA, 20 nt, synthetic construct
  source 1..20: mol_type = other RNA
tcttcgccgcctcccgggtg

SEQ ID NO: 154 - RNA, 20 nt, synthetic construct
  source 1..20: mol_type = other RNA
gaggcggcgaagacgcccac

SEQ ID NO: 155 - RNA, 20 nt, synthetic construct
  source 1..20: mol_type = other RNA
aggcggcgaagacgcccact

SEQ ID NO: 156 - RNA, 20 nt, synthetic construct
  source 1..20: mol_type = other RNA
acgcccactgggaccgcgcc

SEQ ID NO: 157 - RNA, 20 nt, synthetic construct
  source 1..20: mol_type = other RNA
cggccaggcgcggtcccagt

SEQ ID NO: 158 - RNA, 20 nt, synthetic construct
  source 1..20: mol_type = other RNA
acggccaggcgcggtcccag

SEQ ID NO: 159 - RNA, 20 nt, synthetic construct
  source 1..20: mol_type = other RNA
gaccgcgcctggccgttttc

SEQ ID NO: 160 - RNA, 20 nt, synthetic construct
  source 1..20: mol_type = other RNA
accgcgcctggccgttttct

SEQ ID NO: 161 - RNA, 20 nt, synthetic construct
  source 1..20: mol_type = other RNA
gcccagaaaacggccaggcg

SEQ ID NO: 162 - RNA, 20 nt, synthetic construct
  source 1..20: mol_type = other RNA
gacgcgcccagaaaacggcc

SEQ ID NO: 163 - RNA, 20 nt, synthetic construct
  source 1..20: mol_type = other RNA
ggcaggacgcgcccagaaaa

SEQ ID NO: 164 - RNA, 20 nt, synthetic construct
  source 1..20: mol_type = other RNA
ctgggcgcgtcctgccccca

SEQ ID NO: 165 - RNA, 20 nt, synthetic construct
  source 1..20: mol_type = other RNA
gagacagaggccgtgggggc

SEQ ID NO: 166 - RNA, 20 nt, synthetic construct
  source 1..20: mol_type = other RNA
cccacggcctctgtctctta

SEQ ID NO: 167 - RNA, 20 nt, synthetic construct
  source 1..20: mol_type = other RNA
ctaagagacagaggccgtgg

SEQ ID NO: 168 - RNA, 20 nt, synthetic construct
  source 1..20: mol_type = other RNA
cctaagagacagaggccgtg

SEQ ID NO: 169 - RNA, 20 nt, synthetic construct
  source 1..20: mol_type = other RNA
ccctaagagacagaggccgt

SEQ ID NO: 170 - RNA, 20 nt, synthetic construct
  source 1..20: mol_type = other RNA
gccctaagagacagaggccg

SEQ ID NO: 171 - RNA, 20 nt, synthetic construct
  source 1..20: mol_type = other RNA
cctctgtctcttagggcgac

SEQ ID NO: 172 - RNA, 20 nt, synthetic construct
  source 1..20: mol_type = other RNA
ctctgtctcttagggcgact

SEQ ID NO: 173 - RNA, 20 nt, synthetic construct
  source 1..20: mol_type = other RNA
ccagtcgccctaagagacag

SEQ ID NO: 174 - RNA, 20 nt, synthetic construct
  source 1..20: mol_type = other RNA
tctcttagggcgactgggcg

SEQ ID NO: 175 - RNA, 20 nt, synthetic construct
  source 1..20: mol_type = other RNA
actgggcgcggaagaaaagc

SEQ ID NO: 176 - RNA, 20 nt, synthetic construct
  source 1..20: mol_type = other RNA
gaaaagctggagagcccctg

SEQ ID NO: 177 - RNA, 20 nt, synthetic construct
  source 1..20: mol_type = other RNA
aaaagctggagagcccctgc

SEQ ID NO: 178 - RNA, 20 nt, synthetic construct
  source 1..20: mol_type = other RNA
aaagctggagagcccctgcg

SEQ ID NO: 179 - RNA, 20 nt, synthetic construct
  source 1..20: mol_type = other RNA
gctggagagcccctgcgggg

SEQ ID NO: 180 - RNA, 20 nt, synthetic construct
  source 1..20: mol_type = other RNA
gagagcccctgcggggtggc

SEQ ID NO: 181 - RNA, 20 nt, synthetic construct
  source 1..20: mol_type = other RNA
agcccctgcggggtggcagg

SEQ ID NO: 182 - RNA, 20 nt, synthetic construct
  source 1..20: mol_type = other RNA
ccctgcggggtggcaggagg

SEQ ID NO: 183 - RNA, 20 nt, synthetic construct
  source 1..20: mol_type = other RNA
cctgcggggtggcaggagga

SEQ ID NO: 184 - RNA, 20 nt, synthetic construct
  source 1..20: mol_type = other RNA
ctcctcctgccaccccgcag

SEQ ID NO: 185 - RNA, 20 nt, synthetic construct
  source 1..20: mol_type = other RNA
cctcctcctgccaccccgca

SEQ ID NO: 186 - RNA, 20 nt, synthetic construct
  source 1..20: mol_type = other RNA
ccctcctcctgccaccccgc

SEQ ID NO: 187 - RNA, 20 nt, synthetic construct
  source 1..20: mol_type = other RNA
gggtgcctgagtcccgcgag

SEQ ID NO: 188 - RNA, 20 nt, synthetic construct
  source 1..20: mol_type = other RNA
cctgagtcccgcgagaggcc

SEQ ID NO: 189 - RNA, 20 nt, synthetic construct
  source 1..20: mol_type = other RNA
ctgagtcccgcgagaggccc

SEQ ID NO: 190 - RNA, 20 nt, synthetic construct
  source 1..20: mol_type = other RNA
ccgggcctctcgcgggactc

SEQ ID NO: 191 - RNA, 20 nt, synthetic construct
  source 1..20: mol_type = other RNA
tcccgcgagaggcccgggcg

SEQ ID NO: 192 - RNA, 20 nt, synthetic construct
  source 1..20: mol_type = other RNA
tcctcgcccgggcctctcgc

SEQ ID NO: 193 - RNA, 20 nt, synthetic construct
  source 1..20: mol_type = other RNA
ttcctcgcccgggcctctcg

SEQ ID NO: 194 - RNA, 20 nt, synthetic construct
  source 1..20: mol_type = other RNA
gctgcgcatcttcctcgccc

SEQ ID NO: 195 - RNA, 20 nt, synthetic construct
  source 1..20: mol_type = other RNA
ggctgcgcatcttcctcgcc

SEQ ID NO: 196 - RNA, 20 nt, synthetic construct
  source 1..20: mol_type = other RNA
ctgctgatccgcgtcccgcc

SEQ ID NO: 197 - RNA, 20 nt, synthetic construct
  source 1..20: mol_type = other RNA
cgggcgggacgcggatcagc

SEQ ID NO: 198 - RNA, 20 nt, synthetic construct
  source 1..20: mol_type = other RNA
tccgcgtcccgcccggcgcc

SEQ ID NO: 199 - RNA, 20 nt, synthetic construct
  source 1..20: mol_type = other RNA
ccgcgtcccgcccggcgcca

SEQ ID NO: 200 - RNA, 20 nt, synthetic construct
  source 1..20: mol_type = other RNA
ccctggcgccgggcgggacg

SEQ ID NO: 201 - RNA, 20 nt, synthetic construct
  source 1..20: mol_type = other RNA
gagggtccctggcgccgggc

SEQ ID NO: 202 - RNA, 20 nt, synthetic construct
  source 1..20: mol_type = other RNA
cggcgccagggaccctcaga

SEQ ID NO: 203 - RNA, 20 nt, synthetic construct
  source 1..20: mol_type = other RNA
ctctgagggtccctggcgcc

SEQ ID NO: 204 - RNA, 20 nt, synthetic construct
  source 1..20: mol_type = other RNA
cctctgagggtccctggcgc

SEQ ID NO: 205 - RNA, 20 nt, synthetic construct
  source 1..20: mol_type = other RNA
ctcctccctctgagggtccc

SEQ ID NO: 206 - RNA, 20 nt, synthetic construct
  source 1..20: mol_type = other RNA
ttgagctctcctccctctga

SEQ ID NO: 207 - RNA, 20 nt, synthetic construct
  source 1..20: mol_type = other RNA
tttgagctctcctccctctg

SEQ ID NO: 208 - RNA, 20 nt, synthetic construct
  source 1..20: mol_type = other RNA
cctcgccccgcgccttcgcg

SEQ ID NO: 209 - RNA, 20 nt, synthetic construct
  source 1..20: mol_type = other RNA
cctcgcgaaggcgcggggcg

SEQ ID NO: 210 - RNA, 20 nt, synthetic construct
  source 1..20: mol_type = other RNA
ttggtcctcgcgaaggcgcg

SEQ ID NO: 211 - RNA, 20 nt, synthetic construct
  source 1..20: mol_type = other RNA
gttggtcctcgcgaaggcgc

SEQ ID NO: 212 - RNA, 20 nt, synthetic construct
  source 1..20: mol_type = other RNA
ggttggtcctcgcgaaggcg

SEQ ID NO: 213 - RNA, 20 nt, synthetic construct
  source 1..20: mol_type = other RNA
gactgggttggtcctcgcga

SEQ ID NO: 214 - RNA, 20 nt, synthetic construct
  source 1..20: mol_type = other RNA
ggcaggcgcggggactgggt

SEQ ID NO: 215 - RNA, 20 nt, synthetic construct
  source 1..20: mol_type = other RNA
tccccgcgcctgccccagag

SEQ ID NO: 216 - RNA, 20 nt, synthetic construct
  source 1..20: mol_type = other RNA
tctggggcaggcgcggggac

SEQ ID NO: 217 - RNA, 20 nt, synthetic construct
  source 1..20: mol_type = other RNA
gccgctctggggcaggcgcg

SEQ ID NO: 218 - RNA, 20 nt, synthetic construct
  source 1..20: mol_type = other RNA
agccgctctggggcaggcgc

SEQ ID NO: 219 - RNA, 20 nt, synthetic construct
  source 1..20: mol_type = other RNA
aagccgctctggggcaggcg

SEQ ID NO: 220 - RNA, 20 nt, synthetic construct
  source 1..20: mol_type = other RNA
tttctaagccgctctggggc

SEQ ID NO: 221 - RNA, 20 nt, synthetic construct
  source 1..20: mol_type = other RNA
ccagagcggcttagaaactc

SEQ ID NO: 222 - RNA, 20 nt, synthetic construct
  source 1..20: mol_type = other RNA
cagagcggcttagaaactca

SEQ ID NO: 223 - RNA, 20 nt, synthetic construct
  source 1..20: mol_type = other RNA
tgagtttctaagccgctctg

SEQ ID NO: 224 - RNA, 20 nt, synthetic construct
  source 1..20: mol_type = other RNA
ctgagtttctaagccgctct

SEQ ID NO: 225 - RNA, 20 nt, synthetic construct
  source 1..20: mol_type = other RNA
cctgagtttctaagccgctc

SEQ ID NO: 226 - RNA, 20 nt, synthetic construct
  source 1..20: mol_type = other RNA
tcagggcacagtgagagcgc

SEQ ID NO: 227 - RNA, 20 nt, synthetic construct
  source 1..20: mol_type = other RNA
cagggcacagtgagagcgca

SEQ ID NO: 228 - RNA, 20 nt, synthetic construct
  source 1..20: mol_type = other RNA
agagcgcagggcgcctcccg

SEQ ID NO: 229 - RNA, 20 nt, synthetic construct
  source 1..20: mol_type = other RNA
ctcccgaggcttcacaccgc

SEQ ID NO: 230 - RNA, 20 nt, synthetic construct
  source 1..20: mol_type = other RNA
cggcggtgtgaagcctcggg

SEQ ID NO: 231 - RNA, 20 nt, synthetic construct
  source 1..20: mol_type = other RNA
gaggcttcacaccgccggcc

SEQ ID NO: 232 - RNA, 20 nt, synthetic construct
  source 1..20: mol_type = other RNA
ggccggcggtgtgaagcctc

SEQ ID NO: 233 - RNA, 20 nt, synthetic construct
  source 1..20: mol_type = other RNA
cggccggcggtgtgaagcct

SEQ ID NO: 234 - RNA, 20 nt, synthetic construct
  source 1..20: mol_type = other RNA
cacaccgccggccgggccag

SEQ ID NO: 235 - RNA, 20 nt, synthetic construct
  source 1..20: mol_type = other RNA
accgccggccgggccagcgg

SEQ ID NO: 236 - RNA, 20 nt, synthetic construct
  source 1..20: mol_type = other RNA
gcctccgctggcccggccgg

SEQ ID NO: 237 - RNA, 20 nt, synthetic construct
  source 1..20: mol_type = other RNA
acagcctccgctggcccggc

SEQ ID NO: 238 - RNA, 20 nt, synthetic construct
  source 1..20: mol_type = other RNA
gggccagcggaggctgtgac

SEQ ID NO: 239 - RNA, 20 nt, synthetic construct
  source 1..20: mol_type = other RNA
ggtcacagcctccgctggcc

SEQ ID NO: 240 - RNA, 20 nt, synthetic construct
  source 1..20: mol_type = other RNA
gctccggtcacagcctccgc

SEQ ID NO: 241 - RNA, 20 nt, synthetic construct
  source 1..20: mol_type = other RNA
gcggcacagagggggcgctc

SEQ ID NO: 242 - RNA, 20 nt, synthetic construct
  source 1..20: mol_type = other RNA
cctctgtgccgcgcacgccg

SEQ ID NO: 243 - RNA, 20 nt, synthetic construct
  source 1..20: mol_type = other RNA
cggcgtgcgcggcacagagg

SEQ ID NO: 244 - RNA, 20 nt, synthetic construct
  source 1..20: mol_type = other RNA
gcggcgtgcgcggcacagag

SEQ ID NO: 245 - RNA, 20 nt, synthetic construct
  source 1..20: mol_type = other RNA
cgcggcgtgcgcggcacaga

SEQ ID NO: 246 - RNA, 20 nt, synthetic construct
  source 1..20: mol_type = other RNA
ccgcggcgtgcgcggcacag

SEQ ID NO: 247 - RNA, 20 nt, synthetic construct
  source 1..20: mol_type = other RNA
gcgcacgccgcggccgccgc

SEQ ID NO: 248 - RNA, 20 nt, synthetic construct
  source 1..20: mol_type = other RNA
cgcacgccgcggccgccgcc

SEQ ID NO: 249 - RNA, 20 nt, synthetic construct
  source 1..20: mol_type = other RNA
ggcggcggccgcggcgtgcg

SEQ ID NO: 250 - RNA, 20 nt, synthetic construct
  source 1..20: mol_type = other RNA
cgccgcggccgccgccgggt

SEQ ID NO: 251 - RNA, 20 nt, synthetic construct
  source 1..20: mol_type = other RNA
gccgcggccgccgccgggtt

SEQ ID NO: 252 - RNA, 20 nt, synthetic construct
  source 1..20: mol_type = other RNA
ccgcggccgccgccgggttg

SEQ ID NO: 253 - RNA, 20 nt, synthetic construct
  source 1..20: mol_type = other RNA
ggccgccgccgggttggggt

SEQ ID NO: 254 - RNA, 20 nt, synthetic construct
  source 1..20: mol_type = other RNA
ccccaacccggcggcggccg

SEQ ID NO: 255 - RNA, 20 nt, synthetic construct
  source 1..20: mol_type = other RNA
gccgggttggggtaggtgag

SEQ ID NO: 256 - RNA, 20 nt, synthetic construct
  source 1..20: mol_type = other RNA
ccgggttggggtaggtgagc

SEQ ID NO: 257 - RNA, 20 nt, synthetic construct
  source 1..20: mol_type = other RNA
gctcacctaccccaacccgg

SEQ ID NO: 258 - RNA, 20 nt, synthetic construct
  source 1..20: mol_type = other RNA
ggttggggtaggtgagcggg

SEQ ID NO: 259 - RNA, 20 nt, synthetic construct
  source 1..20: mol_type = other RNA
cccgctcacctaccccaacc

SEQ ID NO: 260 - RNA, 20 nt, synthetic construct
  source 1..20: mol_type = other RNA
gggtaggtgagcgggaggct

SEQ ID NO: 261 - RNA, 20 nt, synthetic construct
  source 1..20: mol_type = other RNA
ggtaggtgagcgggaggcta

SEQ ID NO: 262 - RNA, 20 nt, synthetic construct
  source 1..20: mol_type = other RNA
cgggaggctagggtacactt

SEQ ID NO: 263 - RNA, 20 nt, synthetic construct
  source 1..20: mol_type = other RNA
gggaggctagggtacacttc

SEQ ID NO: 264 - RNA, 20 nt, synthetic construct
  source 1..20: mol_type = other RNA
ggaggctagggtacacttcg

SEQ ID NO: 265 - RNA, 20 nt, synthetic construct
  source 1..20: mol_type = other RNA
ggctagggtacacttcgggg

SEQ ID NO: 266 - RNA, 20 nt, synthetic construct
  source 1..20: mol_type = other RNA
gctagggtacacttcggggt

SEQ ID NO: 267 - RNA, 20 nt, synthetic construct
  source 1..20: mol_type = other RNA
ctagggtacacttcggggtg

SEQ ID NO: 268 - RNA, 20 nt, synthetic construct
  source 1..20: mol_type = other RNA
tagggtacacttcggggtgg

SEQ ID NO: 269 - RNA, 20 nt, synthetic construct
  source 1..20: mol_type = other RNA
gtacacttcggggtggggga

SEQ ID NO: 270 - RNA, 20 nt, synthetic construct
  source 1..20: mol_type = other RNA
tacacttcggggtgggggat

SEQ ID NO: 271 - RNA, 20 nt, synthetic construct
  source 1..20: mol_type = other RNA
gtgggggatgggcgcgcaca

SEQ ID NO: 272 - RNA, 20 nt, synthetic construct
  source 1..20: mol_type = other RNA
gcgcgcacatggccgccagc

SEQ ID NO: 273 - RNA, 20 nt, synthetic construct
  source 1..20: mol_type = other RNA
gccagcaggcagagttactc

SEQ ID NO: 274 - RNA, 20 nt, synthetic construct
  source 1..20: mol_type = other RNA
ggagtaactctgcctgctgg

SEQ ID NO: 275 - RNA, 20 nt, synthetic construct
  source 1..20: mol_type = other RNA
accggagtaactctgcctgc

SEQ ID NO: 276 - RNA, 20 nt, synthetic construct
  source 1..20: mol_type = other RNA
gttactccggtaaacacgcc

SEQ ID NO: 277 - RNA, 20 nt, synthetic construct
  source 1..20: mol_type = other RNA
ttactccggtaaacacgcca

SEQ ID NO: 278 - RNA, 20 nt, synthetic construct
  source 1..20: mol_type = other RNA
tccggtaaacacgccaggga

SEQ ID NO: 279 - RNA, 20 nt, synthetic construct
  source 1..20: mol_type = other RNA
ggtaaacacgccagggacgg

SEQ ID NO: 280 - RNA, 20 nt, synthetic construct
  source 1..20: mol_type = other RNA
gccgtccctggcgtgtttac

SEQ ID NO: 281 - RNA, 20 nt, synthetic construct
  source 1..20: mol_type = other RNA
gccagggacggcggcgcgcg

SEQ ID NO: 282 - RNA, 20 nt, synthetic construct
  source 1..20: mol_type = other RNA
ccagggacggcggcgcgcgc

SEQ ID NO: 283 - RNA, 20 nt, synthetic construct
  source 1..20: mol_type = other RNA
gggacggcggcgcgcgcggg

SEQ ID NO: 284 - RNA, 20 nt, synthetic construct
  source 1..20: mol_type = other RNA
cccgcgcgcgccgccgtccc

SEQ ID NO: 285 - RNA, 20 nt, synthetic construct
  source 1..20: mol_type = other RNA
gcgcgcgggaggcaacccag

SEQ ID NO: 286 - RNA, 20 nt, synthetic construct
  source 1..20: mol_type = other RNA
cgcgcgggaggcaacccagc

SEQ ID NO: 287 - RNA, 20 nt, synthetic construct
  source 1..20: mol_type = other RNA
gcgcgggaggcaacccagcg

SEQ ID NO: 288 - RNA, 20 nt, synthetic construct
  source 1..20: mol_type = other RNA
aaggcgggggttgccccgct

SEQ ID NO: 289 - RNA, 20 nt, synthetic construct
  source 1..20: mol_type = other RNA
aaaggcgggggttgccccgc

SEQ ID NO: 290 - RNA, 20 nt, synthetic construct
  source 1..20: mol_type = other RNA
gctcggacaggtaaaggcgg

SEQ ID NO: 291 - RNA, 20 nt, synthetic construct
  source 1..20: mol_type = other RNA
ggctcggacaggtaaaggcg

SEQ ID NO: 292 - RNA, 20 nt, synthetic construct
  source 1..20: mol_type = other RNA
aggctcggacaggtaaaggc

SEQ ID NO: 293 - RNA, 20 nt, synthetic construct
  source 1..20: mol_type = other RNA
caggctcggacaggtaaagg

SEQ ID NO: 294 - RNA, 20 nt, synthetic construct
  source 1..20: mol_type = other RNA
gtgcaggctcggacaggtaa

SEQ ID NO: 295 - RNA, 20 nt, synthetic construct
  source 1..20: mol_type = other RNA
ctgtccgagcctgcacgcgc

SEQ ID NO: 296 - RNA, 20 nt, synthetic construct
  source 1..20: mol_type = other RNA
tccgagcctgcacgcgccgg

SEQ ID NO: 297 - RNA, 20 nt, synthetic construct
  source 1..20: mol_type = other RNA
cggcgcgtgcaggctcggac

SEQ ID NO: 298 - RNA, 20 nt, synthetic construct
  source 1..20: mol_type = other RNA
cctgcacgcgccggcggccg

SEQ ID NO: 299 - RNA, 20 nt, synthetic construct
  source 1..20: mol_type = other RNA
ccgcggccgccggcgcgtgc

SEQ ID NO: 300 - RNA, 20 nt, synthetic construct
  source 1..20: mol_type = other RNA
cgccggcggccgcggcgccg

SEQ ID NO: 301 - RNA, 20 nt, synthetic construct
  source 1..20: mol_type = other RNA
gccggcggccgcggcgccga

SEQ ID NO: 302 - RNA, 20 nt, synthetic construct
  source 1..20: mol_type = other RNA
ccggcggccgcggcgccgag

SEQ ID NO: 303 - RNA, 20 nt, synthetic construct
  source 1..20: mol_type = other RNA
cggcggccgcggcgccgagg

SEQ ID NO: 304 - RNA, 20 nt, synthetic construct
  source 1..20: mol_type = other RNA
ggcggccgcggcgccgaggg

SEQ ID NO: 305 - RNA, 20 nt, synthetic construct
  source 1..20: mol_type = other RNA
ggccgcggcgccgagggggg

SEQ ID NO: 306 - RNA, 20 nt, synthetic construct
  source 1..20: mol_type = other RNA
ctccgcccccctcggcgccg

SEQ ID NO: 307 - RNA, 20 nt, synthetic construct
  source 1..20: mol_type = other RNA
ctggcaagctccgcccccct

SEQ ID NO: 308 - RNA, 20 nt, synthetic construct
  source 1..20: mol_type = other RNA
gagcttgccagcccgcgcgc

SEQ ID NO: 309 - RNA, 20 nt, synthetic construct
  source 1..20: mol_type = other RNA
agcttgccagcccgcgcgcc

SEQ ID NO: 310 - RNA, 20 nt, synthetic construct
  source 1..20: mol_type = other RNA
gcttgccagcccgcgcgccg

SEQ ID NO: 311 - RNA, 20 nt, synthetic construct
  source 1..20: mol_type = other RNA
tgccagcccgcgcgccgggg

SEQ ID NO: 312 - RNA, 20 nt, synthetic construct
  source 1..20: mol_type = other RNA
gccagcccgcgcgccggggc

SEQ ID NO: 313 - RNA, 20 nt, synthetic construct
  source 1..20: mol_type = other RNA
tcccgccccggcgcgcgggc

SEQ ID NO: 314 - RNA, 20 nt, synthetic construct
  source 1..20: mol_type = other RNA
cgcgccggggcgggacctag

SEQ ID NO: 315 - RNA, 20 nt, synthetic construct
  source 1..20: mol_type = other RNA
gcgccggggcgggacctagc

SEQ ID NO: 316 - RNA, 20 nt, synthetic construct
  source 1..20: mol_type = other RNA
cgccggggcgggacctagcg

SEQ ID NO: 317 - RNA, 20 nt, synthetic construct
  source 1..20: mol_type = other RNA
gccggggcgggacctagcgg

SEQ ID NO: 318 - RNA, 20 nt, synthetic construct
  source 1..20: mol_type = other RNA
ggggcgggacctagcggggg

SEQ ID NO: 319 - RNA, 20 nt, synthetic construct
  source 1..20: mol_type = other RNA
gggcgggacctagcgggggc

SEQ ID NO: 320 - RNA, 20 nt, synthetic construct
  source 1..20: mol_type = other RNA
ggcgggacctagcgggggcg

SEQ ID NO: 321 - RNA, 20 nt, synthetic construct
  source 1..20: mol_type = other RNA
gcccccgctaggtcccgccc

SEQ ID NO: 322 - RNA, 20 nt, synthetic construct
  source 1..20: mol_type = other RNA
ctgcggaccccgcccccgct

SEQ ID NO: 323 - RNA, 20 nt, synthetic construct
  source 1..20: mol_type = other RNA
ggggcggggtccgcagtgat

SEQ ID NO: 324 - RNA, 20 nt, synthetic construct
  source 1..20: mol_type = other RNA
gggcggggtccgcagtgatt

SEQ ID NO: 325 - RNA, 20 nt, synthetic construct
  source 1..20: mol_type = other RNA
ggtccgcagtgattgggcgt

SEQ ID NO: 326 - RNA, 20 nt, synthetic construct
  source 1..20: mol_type = other RNA
gcagtgattgggcgtaggag

SEQ ID NO: 327 - RNA, 20 nt, synthetic construct
  source 1..20: mol_type = other RNA
cagtgattgggcgtaggagc

SEQ ID NO: 328 - RNA, 20 nt, synthetic construct
  source 1..20: mol_type = other RNA
agtgattgggcgtaggagcg

SEQ ID NO: 329 - RNA, 20 nt, synthetic construct
  source 1..20: mol_type = other RNA
gctcctacgcccaatcactg

SEQ ID NO: 330 - RNA, 20 nt, synthetic construct
  source 1..20: mol_type = other RNA
gcggggccgccagccagagc

SEQ ID NO: 331 - RNA, 20 nt, synthetic construct
  source 1..20: mol_type = other RNA
cggggccgccagccagagct

SEQ ID NO: 332 - RNA, 20 nt, synthetic construct
  source 1..20: mol_type = other RNA
gccagccagagctgggctgc

SEQ ID NO: 333 - RNA, 20 nt, synthetic construct
  source 1..20: mol_type = other RNA
ccagccagagctgggctgca

SEQ ID NO: 334 - RNA, 20 nt, synthetic construct
  source 1..20: mol_type = other RNA
tgcagcccagctctggctgg

SEQ ID NO: 335 - RNA, 20 nt, synthetic construct
  source 1..20: mol_type = other RNA
ccctgcagcccagctctggc

SEQ ID NO: 336 - RNA, 20 nt, synthetic construct
  source 1..20: mol_type = other RNA
gctgggctgcagggccgcgc

SEQ ID NO: 337 - RNA, 20 nt, synthetic construct
  source 1..20: mol_type = other RNA
ggagcgaagtgaaacctgcg

SEQ ID NO: 338 - RNA, 20 nt, synthetic construct
  source 1..20: mol_type = other RNA
cttcgctccgcgcagccgcc

SEQ ID NO: 339 - RNA, 20 nt, synthetic construct
  source 1..20: mol_type = other RNA
ctgcagaccaggcggctgcg

SEQ ID NO: 340 - RNA, 20 nt, synthetic construct
  source 1..20: mol_type = other RNA
ccgcctggtctgcagtttgt

SEQ ID NO: 341 - RNA, 20 nt, synthetic construct
  source 1..20: mol_type = other RNA
ccaacaaactgcagaccagg

SEQ ID NO: 342 - RNA, 20 nt, synthetic construct
  source 1..20: mol_type = other RNA
gctccaacaaactgcagacc

SEQ ID NO: 343 - RNA, 20 nt, synthetic construct
  source 1..20: mol_type = other RNA
ggcggcagcggcagcggcgc

SEQ ID NO: 344 - RNA, 20 nt, synthetic construct
  source 1..20: mol_type = other RNA
ggcggcggcggcagcggcag

SEQ ID NO: 345 - RNA, 20 nt, synthetic construct
  source 1..20: mol_type = other RNA
ggcggcggcggcggcggcag

SEQ ID NO: 346 - RNA, 20 nt, synthetic construct
  source 1..20: mol_type = other RNA
ggcggcggcggcggcggcgg

SEQ ID NO: 347 - RNA, 20 nt, synthetic construct
  source 1..20: mol_type = other RNA
ggcggcggcggcggcggcgg

SEQ ID NO: 348 - RNA, 20 nt, synthetic construct
  source 1..20: mol_type = other RNA
ggcggcggcggcggcggcgg

SEQ ID NO: 349 - RNA, 20 nt, synthetic construct
  source 1..20: mol_type = other RNA
ggcggcggcggcggcggcgg

SEQ ID NO: 350 - RNA, 20 nt, synthetic construct
  source 1..20: mol_type = other RNA
ggcggcggcggcggcggcgg

SEQ ID NO: 351 - RNA, 20 nt, synthetic construct
  source 1..20: mol_type = other RNA
ggcggcggcggcggcggcgg

SEQ ID NO: 352 - RNA, 20 nt, synthetic construct
  source 1..20: mol_type = other RNA
ggcggcggcggcggcggcgg

SEQ ID NO: 353 - RNA, 20 nt, synthetic construct
  source 1..20: mol_type = other RNA
agtggcggcggcggcggcgg

SEQ ID NO: 354 - RNA, 20 nt, synthetic construct
  source 1..20: mol_type = other RNA
ggtagtggcggcggcggcgg

SEQ ID NO: 355 - RNA, 20 nt, synthetic construct
  source 1..20: mol_type = other RNA
ggtggtagtggcggcggcgg

SEQ ID NO: 356 - RNA, 20 nt, synthetic construct
  source 1..20: mol_type = other RNA
agtggtggtagtggcggcgg

SEQ ID NO: 357 - RNA, 20 nt, synthetic construct
  source 1..20: mol_type = other RNA
tcaagtggtggtagtggcgg

SEQ ID NO: 358 - RNA, 20 nt, synthetic construct
  source 1..20: mol_type = other RNA
gaatcaagtggtggtagtgg

SEQ ID NO: 359 - RNA, 20 nt, synthetic construct
  source 1..20: mol_type = other RNA
caagaatcaagtggtggtag

SEQ ID NO: 360 - RNA, 20 nt, synthetic construct
  source 1..20: mol_type = other RNA
tggctgcaagaatcaagtgg

SEQ ID NO: 361 - RNA, 20 nt, synthetic construct
  source 1..20: mol_type = other RNA
gggtggctgcaagaatcaag

SEQ ID NO: 362 - RNA, 20 nt, synthetic construct
  source 1..20: mol_type = other RNA
gtgtggcagggttcgcaggg

SEQ ID NO: 363 - RNA, 20 nt, synthetic construct
  source 1..20: mol_type = other RNA
gcagtgtggcagggttcgca

SEQ ID NO: 364 - RNA, 20 nt, synthetic construct
  source 1..20: mol_type = other RNA
cgcagtgtggcagggttcgc

SEQ ID NO: 365 - RNA, 20 nt, synthetic construct
  source 1..20: mol_type = other RNA
gatgcgatcgcagtgtggca

SEQ ID NO: 366 - RNA, 20 nt, synthetic construct
  source 1..20: mol_type = other RNA
tgatgcgatcgcagtgtggc

SEQ ID NO: 367 - RNA, 20 nt, synthetic construct
  source 1..20: mol_type = other RNA
acactgcgatcgcatcatcg

SEQ ID NO: 368 - RNA, 20 nt, synthetic construct
  source 1..20: mol_type = other RNA
gcgatgatgcgatcgcagtg

SEQ ID NO: 369 - RNA, 20 nt, synthetic construct
  source 1..20: mol_type = other RNA
gatcgcatcatcgcggtatt

SEQ ID NO: 370 - RNA, 20 nt, synthetic construct
  source 1..20: mol_type = other RNA
cgttcccgccgccaccgcct

SEQ ID NO: 371 - RNA, 20 nt, synthetic construct
  source 1..20: mol_type = other RNA
ggcgccgaggcggtggcggc

SEQ ID NO: 372 - RNA, 20 nt, synthetic construct
  source 1..20: mol_type = other RNA
gggcgccgaggcggtggcgg

SEQ ID NO: 373 - RNA, 20 nt, synthetic construct
  source 1..20: mol_type = other RNA
aaagggcgccgaggcggtgg

SEQ ID NO: 374 - RNA, 20 nt, synthetic construct
  source 1..20: mol_type = other RNA
aagaaagggcgccgaggcgg

SEQ ID NO: 375 - RNA, 20 nt, synthetic construct
  source 1..20: mol_type = other RNA
gccaagaaagggcgccgagg

SEQ ID NO: 376 - RNA, 20 nt, synthetic construct
  source 1..20: mol_type = other RNA
agggccaagaaagggcgccg

SEQ ID NO: 377 - RNA, 20 nt, synthetic construct
  source 1..20: mol_type = other RNA
ggggaacaagggccaagaaa

SEQ ID NO: 378 - RNA, 20 nt, synthetic construct
  source 1..20: mol_type = other RNA
gggggaacaagggccaagaa

SEQ ID NO: 379 - RNA, 20 nt, synthetic construct
  source 1..20: mol_type = other RNA
tcagacatttgggggaacaa

SEQ ID NO: 380 - RNA, 20 nt, synthetic construct
  source 1..20: mol_type = other RNA
gtcagacatttgggggaaca

SEQ ID NO: 381 - RNA, 20 nt, synthetic construct
  source 1..20: mol_type = other RNA
aaatgtctgactctgactct

SEQ ID NO: 382 - RNA, 20 nt, synthetic construct
  source 1..20: mol_type = other RNA
gagtcagagtcagacatttg

SEQ ID NO: 383 - RNA, 20 nt, synthetic construct
  source 1..20: mol_type = other RNA
agagtcagagtcagacattt

SEQ ID NO: 384 - RNA, 20 nt, synthetic construct
  source 1..20: mol_type = other RNA
gagagtcagagtcagacatt

SEQ ID NO: 385 - RNA, 20 nt, synthetic construct
  source 1..20: mol_type = other RNA
ctctcggactgagaaacgca

SEQ ID NO: 386 - RNA, 20 nt, synthetic construct
  source 1..20: mol_type = other RNA
aggtaaatacctccaaatcc

SEQ ID NO: 387 - RNA, 20 nt, synthetic construct
  source 1..20: mol_type = other RNA
ggtaaatacctccaaatccc

SEQ ID NO: 388 - RNA, 20 nt, synthetic construct
  source 1..20: mol_type = other RNA
gtaaatacctccaaatcccg

SEQ ID NO: 389 - RNA, 20 nt, synthetic construct
  source 1..20: mol_type = other RNA
tacctccaaatcccggggcg

SEQ ID NO: 390 - RNA, 20 nt, synthetic construct
  source 1..20: mol_type = other RNA
acctccaaatcccggggcgc

SEQ ID NO: 391 - RNA, 20 nt, synthetic construct
  source 1..20: mol_type = other RNA
caaatcccggggcgcgggcc

SEQ ID NO: 392 - RNA, 20 nt, synthetic construct
  source 1..20: mol_type = other RNA
gcccgcgccccgggatttgg

SEQ ID NO: 393 - RNA, 20 nt, synthetic construct
  source 1..20: mol_type = other RNA
caggcccgcgccccgggatt

SEQ ID NO: 394 - RNA, 20 nt, synthetic construct
  source 1..20: mol_type = other RNA
gggcgcgggcctggcaccga

SEQ ID NO: 395 - RNA, 20 nt, synthetic construct
  source 1..20: mol_type = other RNA
cggtgccaggcccgcgcccc

SEQ ID NO: 396 - RNA, 20 nt, synthetic construct
  source 1..20: mol_type = other RNA
tcggtgccaggcccgcgccc

SEQ ID NO: 397 - RNA, 20 nt, synthetic construct
  source 1..20: mol_type = other RNA
gctagtcttccttcggtgcc

SEQ ID NO: 398 - RNA, 20 nt, synthetic construct
  source 1..20: mol_type = other RNA
ctccagcgctagtcttcctt

SEQ ID NO: 399 - RNA, 20 nt, synthetic construct
  source 1..20: mol_type = other RNA
gactagcgctggagcccgaa

SEQ ID NO: 400 - RNA, 20 nt, synthetic construct
  source 1..20: mol_type = other RNA
ggcagtaggtggtgccgttc

SEQ ID NO: 401 - RNA, 20 nt, synthetic construct
  source 1..20: mol_type = other RNA
gggcagtaggtggtgccgtt

SEQ ID NO: 402 - RNA, 20 nt, synthetic construct
  source 1..20: mol_type = other RNA
cacgggaagcgggcagtagg

SEQ ID NO: 403 - RNA, 20 nt, synthetic construct
  source 1..20: mol_type = other RNA
gtgcacgggaagcgggcagt

SEQ ID NO: 404 - RNA, 20 nt, synthetic construct
  source 1..20: mol_type = other RNA
gcttcccgtgcacgtgcgag

SEQ ID NO: 405 - RNA, 20 nt, synthetic construct
  source 1..20: mol_type = other RNA
ctcgcacgtgcacgggaagc

SEQ ID NO: 406 - RNA, 20 nt, synthetic construct
  source 1..20: mol_type = other RNA
gctcgcacgtgcacgggaag

SEQ ID NO: 407 - RNA, 20 nt, synthetic construct
  source 1..20: mol_type = other RNA
gtctccgctcgcacgtgcac

SEQ ID NO: 408 - RNA, 20 nt, synthetic construct
  source 1..20: mol_type = other RNA
cgtctccgctcgcacgtgca

SEQ ID NO: 409 - RNA, 20 nt, synthetic construct
  source 1..20: mol_type = other RNA
gcgagcggagacgcttgcat

SEQ ID NO: 410 - RNA, 20 nt, synthetic construct
  source 1..20: mol_type = other RNA
gcatcggcgccgcttgtcgc

SEQ ID NO: 411 - RNA, 20 nt, synthetic construct
  source 1..20: mol_type = other RNA
tcggcgccgcttgtcgccgg

SEQ ID NO: 412 - RNA, 20 nt, synthetic construct
  source 1..20: mol_type = other RNA
cggcgccgcttgtcgccggc

SEQ ID NO: 413 - RNA, 20 nt, synthetic construct
  source 1..20: mol_type = other RNA
cgccgcttgtcgccggcggg

SEQ ID NO: 414 - RNA, 20 nt, synthetic construct
  source 1..20: mol_type = other RNA
cgcttgtcgccggcgggagg

SEQ ID NO: 415 - RNA, 20 nt, synthetic construct
  source 1..20: mol_type = other RNA
gcttgtcgccggcgggaggt

SEQ ID NO: 416 - RNA, 20 nt, synthetic construct
  source 1..20: mol_type = other RNA
cttgtcgccggcgggaggtg

SEQ ID NO: 417 - RNA, 20 nt, synthetic construct
  source 1..20: mol_type = other RNA
cacctcccgccggcgacaag

SEQ ID NO: 418 - RNA, 20 nt, synthetic construct
  source 1..20: mol_type = other RNA
gcgggaggtggggatccgtg

SEQ ID NO: 419 - RNA, 20 nt, synthetic construct
  source 1..20: mol_type = other RNA
cacggatccccacctcccgc

SEQ ID NO: 420 - RNA, 20 nt, synthetic construct
  source 1..20: mol_type = other RNA
aggtggggatccgtgtggat

SEQ ID NO: 421 - RNA, 20 nt, synthetic construct
  source 1..20: mol_type = other RNA
ggtggggatccgtgtggatc

SEQ ID NO: 422 - RNA, 20 nt, synthetic construct
  source 1..20: mol_type = other RNA
gtgtggatcgggttccctct

SEQ ID NO: 423 - RNA, 20 nt, synthetic construct
  source 1..20: mol_type = other RNA
tgtggatcgggttccctctc

SEQ ID NO: 424 - RNA, 20 nt, synthetic construct
  source 1..20: mol_type = other RNA
gagagggaacccgatccaca

SEQ ID NO: 425 - RNA, 20 nt, synthetic construct
  source 1..20: mol_type = other RNA
gatcgggttccctctcgggc

SEQ ID NO: 426 - RNA, 20 nt, synthetic construct
  source 1..20: mol_type = other RNA
taaagagaacctgcccgaga

SEQ ID NO: 427 - RNA, 20 nt, synthetic construct
  source 1..20: mol_type = other RNA
ttaaagagaacctgcccgag

SEQ ID NO: 428 - RNA, 20 nt, synthetic construct
  source 1..20: mol_type = other RNA
ttaaagaaaagtcgttcacg

SEQ ID NO: 429 - RNA, 20 nt, synthetic construct
  source 1..20: mol_type = other RNA
gtcgttcacgcggaacctgc

SEQ ID NO: 430 - RNA, 20 nt, synthetic construct
  source 1..20: mol_type = other RNA
acgcggaacctgcaggctct

SEQ ID NO: 431 - RNA, 20 nt, synthetic construct
  source 1..20: mol_type = other RNA
gcaggctcttggccgaagtg

SEQ ID NO: 432 - RNA, 20 nt, synthetic construct
  source 1..20: mol_type = other RNA
cacttcggccaagagcctgc

SEQ ID NO: 433 - RNA, 20 nt, synthetic construct
  source 1..20: mol_type = other RNA
ctcttggccgaagtgcggct

SEQ ID NO: 434 - RNA, 20 nt, synthetic construct
  source 1..20: mol_type = other RNA
tcttggccgaagtgcggctt

SEQ ID NO: 435 - RNA, 20 nt, synthetic construct
  source 1..20: mol_type = other RNA
ggccgaagtgcggcttggga

SEQ ID NO: 436 - RNA, 20 nt, synthetic construct
  source 1..20: mol_type = other RNA
gccgaagtgcggcttgggac

SEQ ID NO: 437 - RNA, 20 nt, synthetic construct
  source 1..20: mol_type = other RNA
tcccgtcccaagccgcactt

SEQ ID NO: 438 - RNA, 20 nt, synthetic construct
  source 1..20: mol_type = other RNA
ttgggacgggatgctgcgcg

SEQ ID NO: 439 - RNA, 20 nt, synthetic construct
  source 1..20: mol_type = other RNA
tgggacgggatgctgcgcgc

SEQ ID NO: 440 - RNA, 20 nt, synthetic construct
  source 1..20: mol_type = other RNA
cgggatgctgcgcgcgggcc

SEQ ID NO: 441 - RNA, 20 nt, synthetic construct
  source 1..20: mol_type = other RNA
gctgcgcgcgggcctggtga

SEQ ID NO: 442 - RNA, 20 nt, synthetic construct
  source 1..20: mol_type = other RNA
ctgcgcgcgggcctggtgaa

SEQ ID NO: 443 - RNA, 20 nt, synthetic construct
  source 1..20: mol_type = other RNA
cgggcctggtgaagggtcgt

SEQ ID NO: 444 - RNA, 20 nt, synthetic construct
  source 1..20: mol_type = other RNA
ctggtgaagggtcgtaggtc

SEQ ID NO: 445 - RNA, 20 nt, synthetic construct
  source 1..20: mol_type = other RNA
tggtgaagggtcgtaggtcc

SEQ ID NO: 446 - RNA, 20 nt, synthetic construct
  source 1..20: mol_type = other RNA
cggacctacgacccttcacc

SEQ ID NO: 447 - RNA, 20 nt, synthetic construct
  source 1..20: mol_type = other RNA
gaagggtcgtaggtccgggc

SEQ ID NO: 448 - RNA, 20 nt, synthetic construct
  source 1..20: mol_type = other RNA
gggtcgtaggtccgggcagg

SEQ ID NO: 449 - RNA, 20 nt, synthetic construct
  source 1..20: mol_type = other RNA
gtaggtccgggcaggaggag

SEQ ID NO: 450 - RNA, 20 nt, synthetic construct
  source 1..20: mol_type = other RNA
gcgctgcctctcctcctgcc

SEQ ID NO: 451 - RNA, 20 nt, synthetic construct
  source 1..20: mol_type = other RNA
gagaggcagcgcgtgccttt

SEQ ID NO: 452 - RNA, 20 nt, synthetic construct
  source 1..20: mol_type = other RNA
cagcgcgtgcctttcggcgc

SEQ ID NO: 453 - RNA, 20 nt, synthetic construct
  source 1..20: mol_type = other RNA
cgtgcctttcggcgccggcc

SEQ ID NO: 454 - RNA, 20 nt, synthetic construct
  source 1..20: mol_type = other RNA
gtgcctttcggcgccggccc

SEQ ID NO: 455 - RNA, 20 nt, synthetic construct
  source 1..20: mol_type = other RNA
gctcccgggccggcgccgaa

SEQ ID NO: 456 - RNA, 20 nt, synthetic construct
  source 1..20: mol_type = other RNA
caggtcctcagctcccgggc

SEQ ID NO: 457 - RNA, 20 nt, synthetic construct
  source 1..20: mol_type = other RNA
cgagcaggtcctcagctccc

SEQ ID NO: 458 - RNA, 20 nt, synthetic construct
  source 1..20: mol_type = other RNA
acgagcaggtcctcagctcc

SEQ ID NO: 459 - RNA, 20 nt, synthetic construct
  source 1..20: mol_type = other RNA
tgaggacctgctcgtagtat

SEQ ID NO: 460 - RNA, 20 nt, synthetic construct
  source 1..20: mol_type = other RNA
gaggacctgctcgtagtatc

SEQ ID NO: 461 - RNA, 20 nt, synthetic construct
  source 1..20: mol_type = other RNA
cacagcccgatactacgagc

SEQ ID NO: 462 - RNA, 20 nt, synthetic construct
  source 1..20: mol_type = other RNA
tatcgggctgtgcgcccagc

SEQ ID NO: 463 - RNA, 20 nt, synthetic construct
  source 1..20: mol_type = other RNA
cagctggaaagtctcgccgc

SEQ ID NO: 464 - RNA, 20 nt, synthetic construct
  source 1..20: mol_type = other RNA
ggcggcgagactttccagct

SEQ ID NO: 465 - RNA, 20 nt, synthetic construct
  source 1..20: mol_type = other RNA
cggcggcgagactttccagc

SEQ ID NO: 466 - RNA, 20 nt, synthetic construct
  source 1..20: mol_type = other RNA
gaaagtctcgccgccggctc

SEQ ID NO: 467 - RNA, 20 nt, synthetic construct
  source 1..20: mol_type = other RNA
tctgagggcgccggagccgg

SEQ ID NO: 468 - RNA, 20 nt, synthetic construct
  source 1..20: mol_type = other RNA
ctccggcgccctcagagtag

SEQ ID NO: 469 - RNA, 20 nt, synthetic construct
  source 1..20: mol_type = other RNA
tactctgagggcgccggagc

SEQ ID NO: 470 - RNA, 20 nt, synthetic construct
  source 1..20: mol_type = other RNA
ggccgctactctgagggcgc

SEQ ID NO: 471 - RNA, 20 nt, synthetic construct
  source 1..20: mol_type = other RNA
ctgcgcggccgctactctga

SEQ ID NO: 472 - RNA, 20 nt, synthetic construct
  source 1..20: mol_type = other RNA
actgcgcggccgctactctg

SEQ ID NO: 473 - RNA, 20 nt, synthetic construct
  source 1..20: mol_type = other RNA
agtagcggccgcgcagtgtg

SEQ ID NO: 474 - RNA, 20 nt, synthetic construct
  source 1..20: mol_type = other RNA
gtagcggccgcgcagtgtga

SEQ ID NO: 475 - RNA, 20 nt, synthetic construct
  source 1..20: mol_type = other RNA
cgaaacaccctcacactgcg

SEQ ID NO: 476 - RNA, 20 nt, synthetic construct
  source 1..20: mol_type = other RNA
tgtgagggtgtttcgtgtct

SEQ ID NO: 477 - RNA, 20 nt, synthetic construct
  source 1..20: mol_type = other RNA
tgtttcgtgtcttggttttt

SEQ ID NO: 478 - RNA, 20 nt, synthetic construct
  source 1..20: mol_type = other RNA
gtttcgtgtcttggtttttt

SEQ ID NO: 479 - RNA, 20 nt, synthetic construct
  source 1..20: mol_type = other RNA
tttcgtgtcttggttttttg

SEQ ID NO: 480 - RNA, 20 nt, synthetic construct
  source 1..20: mol_type = other RNA
tcttggttttttggggcgcg

SEQ ID NO: 481 - RNA, 20 nt, synthetic construct
  source 1..20: mol_type = other RNA
cttggttttttggggcgcgt

SEQ ID NO: 482 - RNA, 20 nt, synthetic construct
  source 1..20: mol_type = other RNA
tggggcgcgtgggcctgttg

SEQ ID NO: 483 - RNA, 20 nt, synthetic construct
  source 1..20: mol_type = other RNA
ggcgcgtgggcctgttgcgg

SEQ ID NO: 484 - RNA, 20 nt, synthetic construct
  source 1..20: mol_type = other RNA
ggcctgttgcggaggatttg

SEQ ID NO: 485 - RNA, 20 nt, synthetic construct
  source 1..20: mol_type = other RNA
ttccgcaaatcctccgcaac

SEQ ID NO: 486 - RNA, 20 nt, synthetic construct
  source 1..20: mol_type = other RNA
gcggaggatttgcggaactg

SEQ ID NO: 487 - RNA, 20 nt, synthetic construct
  source 1..20: mol_type = other RNA
gaggatttgcggaactgcgg

SEQ ID NO: 488 - RNA, 20 nt, synthetic construct
  source 1..20: mol_type = other RNA
gtgatttaactgacgagaca

SEQ ID NO: 489 - RNA, 20 nt, synthetic construct
  source 1..20: mol_type = other RNA
gcttttccttttactcattc

SEQ ID NO: 490 - RNA, 20 nt, synthetic construct
  source 1..20: mol_type = other RNA
ccttttactcattcaggcca

SEQ ID NO: 491 - RNA, 20 nt, synthetic construct
  source 1..20: mol_type = other RNA
ccttggcctgaatgagtaaa

SEQ ID NO: 492 - RNA, 20 nt, synthetic construct
  source 1..20: mol_type = other RNA
actcattcaggccaaggttt

SEQ ID NO: 493 - RNA, 20 nt, synthetic construct
  source 1..20: mol_type = other RNA
ctcattcaggccaaggtttc

SEQ ID NO: 494 - RNA, 20 nt, synthetic construct
  source 1..20: mol_type = other RNA
tcattcaggccaaggtttcg

SEQ ID NO: 495 - RNA, 20 nt, synthetic construct
  source 1..20: mol_type = other RNA
cagcagtggccccgaaacct

SEQ ID NO: 496 - RNA, 20 nt, synthetic construct
  source 1..20: mol_type = other RNA
tgagaaagcgaacgcagcag

SEQ ID NO: 497 - RNA, 20 nt, synthetic construct
  source 1..20: mol_type = other RNA
ttcgctttctcaagcgtacc

SEQ ID NO: 498 - RNA, 20 nt, synthetic construct
  source 1..20: mol_type = other RNA
tcgctttctcaagcgtacct

SEQ ID NO: 499 - RNA, 20 nt, synthetic construct
  source 1..20: mol_type = other RNA
cgctttctcaagcgtacctg

SEQ ID NO: 500 - RNA, 20 nt, synthetic construct
  source 1..20: mol_type = other RNA
ggggcccctgcttgctctgc

SEQ ID NO: 501 - RNA, 20 nt, synthetic construct
  source 1..20: mol_type = other RNA
gcagagcaagcaggggcccc

SEQ ID NO: 502 - RNA, 20 nt, synthetic construct
  source 1..20: mol_type = other RNA
gactcctgcagagcaagcag

SEQ ID NO: 503 - RNA, 20 nt, synthetic construct
  source 1..20: mol_type = other RNA
ggactcctgcagagcaagca

SEQ ID NO: 504 - RNA, 20 nt, synthetic construct
  source 1..20: mol_type = other RNA
aggactcctgcagagcaagc

SEQ ID NO: 505 - RNA, 20 nt, synthetic construct
  source 1..20: mol_type = other RNA
gtgcggatggcacaggccgc

SEQ ID NO: 506 - RNA, 20 nt, synthetic construct
  source 1..20: mol_type = other RNA
gtgccatccgcacgattccc

SEQ ID NO: 507 - RNA, 20 nt, synthetic construct
  source 1..20: mol_type = other RNA
gggaatcgtgcggatggcac

SEQ ID NO: 508 - RNA, 20 nt, synthetic construct
  source 1..20: mol_type = other RNA
ctgccagggaatcgtgcgga

SEQ ID NO: 509 - RNA, 20 nt, synthetic construct
  source 1..20: mol_type = other RNA
ctcgctgccagggaatcgtg

SEQ ID NO: 510 - RNA, 20 nt, synthetic construct
  source 1..20: mol_type = other RNA
tccctggcagcgagaaatct

SEQ ID NO: 511 - RNA, 20 nt, synthetic construct
  source 1..20: mol_type = other RNA
acctagatttctcgctgcca

SEQ ID NO: 512 - RNA, 20 nt, synthetic construct
  source 1..20: mol_type = other RNA
gacctagatttctcgctgcc

SEQ ID NO: 513 - RNA, 20 nt, synthetic construct
  source 1..20: mol_type = other RNA
taggtcctcccctgaccacc

SEQ ID NO: 514 - RNA, 20 nt, synthetic construct
  source 1..20: mol_type = other RNA
gcggtccaggtggtcagggg

SEQ ID NO: 515 - RNA, 20 nt, synthetic construct
  source 1..20: mol_type = other RNA
ctgaccacctggaccgcgca

SEQ ID NO: 516 - RNA, 20 nt, synthetic construct
  source 1..20: mol_type = other RNA
tgaccacctggaccgcgcag

SEQ ID NO: 517 - RNA, 20 nt, synthetic construct
  source 1..20: mol_type = other RNA
tgcgcggtccaggtggtcag

SEQ ID NO: 518 - RNA, 20 nt, synthetic construct
  source 1..20: mol_type = other RNA
ctgcgcggtccaggtggtca

SEQ ID NO: 519 - RNA, 20 nt, synthetic construct
  source 1..20: mol_type = other RNA
cctgcgcggtccaggtggtc

SEQ ID NO: 520 - RNA, 20 nt, synthetic construct
  source 1..20: mol_type = other RNA
agtcccctgcgcggtccagg

SEQ ID NO: 521 - RNA, 20 nt, synthetic construct
  source 1..20: mol_type = other RNA
actagtcccctgcgcggtcc

SEQ ID NO: 522 - RNA, 20 nt, synthetic construct
  source 1..20: mol_type = other RNA
cgcaggggactagtcgcggc

SEQ ID NO: 523 - RNA, 20 nt, synthetic construct
  source 1..20: mol_type = other RNA
gccgcgactagtcccctgcg

SEQ ID NO: 524 - RNA, 20 nt, synthetic construct
  source 1..20: mol_type = other RNA
cgcggccggcagaacctgct

SEQ ID NO: 525 - RNA, 20 nt, synthetic construct
  source 1..20: mol_type = other RNA
ggcagaacctgctcggtccc

SEQ ID NO: 526 - RNA, 20 nt, synthetic construct
  source 1..20: mol_type = other RNA
gcagaacctgctcggtccct

SEQ ID NO: 527 - RNA, 20 nt, synthetic construct
  source 1..20: mol_type = other RNA
agggaccgagcaggttctgc

SEQ ID NO: 528 - RNA, 20 nt, synthetic construct
  source 1..20: mol_type = other RNA
aacctgctcggtccctgggc

SEQ ID NO: 529 - RNA, 20 nt, synthetic construct
  source 1..20: mol_type = other RNA
acctgctcggtccctgggcc

SEQ ID NO: 530 - RNA, 20 nt, synthetic construct
  source 1..20: mol_type = other RNA
gcccggcccagggaccgagc

SEQ ID NO: 531 - RNA, 20 nt, synthetic construct
  source 1..20: mol_type = other RNA
cctgggccgggctatcttag

SEQ ID NO: 532 - RNA, 20 nt, synthetic construct
  source 1..20: mol_type = other RNA
cgctaagatagcccggccca

SEQ ID NO: 533 - RNA, 20 nt, synthetic construct
  source 1..20: mol_type = other RNA
ccgctaagatagcccggccc

SEQ ID NO: 534 - RNA, 20 nt, synthetic construct
  source 1..20: mol_type = other RNA
cgtgagccgctaagatagcc

SEQ ID NO: 535 - RNA, 20 nt, synthetic construct
  source 1..20: mol_type = other RNA
atgcccgagcacacccgacc

SEQ ID NO: 536 - RNA, 20 nt, synthetic construct
  source 1..20: mol_type = other RNA
agcacacccgacccggttcg

SEQ ID NO: 537 - RNA, 20 nt, synthetic construct
  source 1..20: mol_type = other RNA
gaaccgggtcgggtgtgctc

SEQ ID NO: 538 - RNA, 20 nt, synthetic construct
  source 1..20: mol_type = other RNA
cgaaccgggtcgggtgtgct

SEQ ID NO: 539 - RNA, 20 nt, synthetic construct
  source 1..20: mol_type = other RNA
cccgacccggttcgcggtgc

SEQ ID NO: 540 - RNA, 20 nt, synthetic construct
  source 1..20: mol_type = other RNA
acccggttcgcggtgcaggc

SEQ ID NO: 541 - RNA, 20 nt, synthetic construct
  source 1..20: mol_type = other RNA
cctgcaccgcgaaccgggtc

SEQ ID NO: 542 - RNA, 20 nt, synthetic construct
  source 1..20: mol_type = other RNA
gcctgcaccgcgaaccgggt

SEQ ID NO: 543 - RNA, 20 nt, synthetic construct
  source 1..20: mol_type = other RNA
cggttcgcggtgcaggctgg

SEQ ID NO: 544 - RNA, 20 nt, synthetic construct
  source 1..20: mol_type = other RNA
gccagcctgcaccgcgaacc

SEQ ID NO: 545 - RNA, 20 nt, synthetic construct
  source 1..20: mol_type = other RNA
cgccagcctgcaccgcgaac

SEQ ID NO: 546 - RNA, 20 nt, synthetic construct
  source 1..20: mol_type = other RNA
gctggcggcgccgtgccctc

SEQ ID NO: 547 - RNA, 20 nt, synthetic construct
  source 1..20: mol_type = other RNA
ctggcggcgccgtgccctct

SEQ ID NO: 548 - RNA, 20 nt, synthetic construct
  source 1..20: mol_type = other RNA
gcaacaggtcccagagggca

SEQ ID NO: 549 - RNA, 20 nt, synthetic construct
  source 1..20: mol_type = other RNA
cctctgggacctgttgcccc

SEQ ID NO: 550 - RNA, 20 nt, synthetic construct
  source 1..20: mol_type = other RNA
ctctgggacctgttgcccca

SEQ ID NO: 551 - RNA, 20 nt, synthetic construct
  source 1..20: mol_type = other RNA
ctggggcaacaggtcccaga

SEQ ID NO: 552 - RNA, 20 nt, synthetic construct
  source 1..20: mol_type = other RNA
gggacctgttgccccagggt

SEQ ID NO: 553 - RNA, 20 nt, synthetic construct
  source 1..20: mol_type = other RNA
tgccccagggttggcgctgc

SEQ ID NO: 554 - RNA, 20 nt, synthetic construct
  source 1..20: mol_type = other RNA
cccagggttggcgctgctgg

SEQ ID NO: 555 - RNA, 20 nt, synthetic construct
  source 1..20: mol_type = other RNA
agggttggcgctgctggtgg

SEQ ID NO: 556 - RNA, 20 nt, synthetic construct
  source 1..20: mol_type = other RNA
caccagcagcgccaaccctg

SEQ ID NO: 557 - RNA, 20 nt, synthetic construct
  source 1..20: mol_type = other RNA
ccaccagcagcgccaaccct

SEQ ID NO: 558 - RNA, 20 nt, synthetic construct
  source 1..20: mol_type = other RNA
tccaccagcagcgccaaccc

SEQ ID NO: 559 - RNA, 20 nt, synthetic construct
  source 1..20: mol_type = other RNA
gctgctggtggagggcccga

SEQ ID NO: 560 - RNA, 20 nt, synthetic construct
  source 1..20: mol_type = other RNA
tggagggcccgacggacgcc

SEQ ID NO: 561 - RNA, 20 nt, synthetic construct
  source 1..20: mol_type = other RNA
ggagggcccgacggacgcca

SEQ ID NO: 562 - RNA, 20 nt, synthetic construct
  source 1..20: mol_type = other RNA
gggcccgacggacgccaggg

SEQ ID NO: 563 - RNA, 20 nt, synthetic construct
  source 1..20: mol_type = other RNA
cccgacggacgccagggcgg

SEQ ID NO: 564 - RNA, 20 nt, synthetic construct
  source 1..20: mol_type = other RNA
ccgacggacgccagggcgga

SEQ ID NO: 565 - RNA, 20 nt, synthetic construct
  source 1..20: mol_type = other RNA
cctccgccctggcgtccgtc

SEQ ID NO: 566 - RNA, 20 nt, synthetic construct
  source 1..20: mol_type = other RNA
ccctccgccctggcgtccgt

SEQ ID NO: 567 - RNA, 20 nt, synthetic construct
  source 1..20: mol_type = other RNA
taaattcacaccctccgccc

SEQ ID NO: 568 - RNA, 20 nt, synthetic construct
  source 1..20: mol_type = other RNA
gagggtgtgaatttactcga

SEQ ID NO: 569 - RNA, 20 nt, synthetic construct
  source 1..20: mol_type = other RNA
gtgaatttactcgatggtcg

SEQ ID NO: 570 - RNA, 20 nt, synthetic construct
  source 1..20: mol_type = other RNA
gtcgcggacgtgcgcgtccg

SEQ ID NO: 571 - RNA, 20 nt, synthetic construct
  source 1..20: mol_type = other RNA
ggacgtgcgcgtccgcggcc

SEQ ID NO: 572 - RNA, 20 nt, synthetic construct
  source 1..20: mol_type = other RNA
gacgtgcgcgtccgcggcca

SEQ ID NO: 573 - RNA, 20 nt, synthetic construct
  source 1..20: mol_type = other RNA
acgtgcgcgtccgcggccag

SEQ ID NO: 574 - RNA, 20 nt, synthetic construct
  source 1..20: mol_type = other RNA
tgcgcgtccgcggccagggg

SEQ ID NO: 575 - RNA, 20 nt, synthetic construct
  source 1..20: mol_type = other RNA
cgcggccaggggtggctctt

SEQ ID NO: 576 - RNA, 20 nt, synthetic construct
  source 1..20: mol_type = other RNA
cgaagagccacccctggccg

SEQ ID NO: 577 - RNA, 20 nt, synthetic construct
  source 1..20: mol_type = other RNA
caaagccgaagagccacccc

SEQ ID NO: 578 - RNA, 20 nt, synthetic construct
  source 1..20: mol_type = other RNA
tcggctttgactcgtgtctg

SEQ ID NO: 579 - RNA, 20 nt, synthetic construct
  source 1..20: mol_type = other RNA
actcgtgtctgcggcgcacc

SEQ ID NO: 580 - RNA, 20 nt, synthetic construct
  source 1..20: mol_type = other RNA
tgcggcgcaccaggagagag

SEQ ID NO: 581 - RNA, 20 nt, synthetic construct
  source 1..20: mol_type = other RNA
caggagagagaggaagttgt

SEQ ID NO: 582 - RNA, 20 nt, synthetic construct
  source 1..20: mol_type = other RNA
gagagagaggaagttgttgg

SEQ ID NO: 583 - RNA, 20 nt, synthetic construct
  source 1..20: mol_type = other RNA
caacaacttcctctctctcc

SEQ ID NO: 584 - RNA, 20 nt, synthetic construct
  source 1..20: mol_type = other RNA
ggagaatagttgccacagcc

SEQ ID NO: 585 - RNA, 20 nt, synthetic construct
  source 1..20: mol_type = other RNA
gagaatagttgccacagcca

SEQ ID NO: 586 - RNA, 20 nt, synthetic construct
  source 1..20: mol_type = other RNA
aatagttgccacagccaggg

SEQ ID NO: 587 - RNA, 20 nt, synthetic construct
  source 1..20: mol_type = other RNA
tgccacagccagggcggtga

SEQ ID NO: 588 - RNA, 20 nt, synthetic construct
  source 1..20: mol_type = other RNA
ggccgtcaccgccctggctg

SEQ ID NO: 589 - RNA, 20 nt, synthetic construct
  source 1..20: mol_type = other RNA
ccagggcggtgacggccgtt

SEQ ID NO: 590 - RNA, 20 nt, synthetic construct
  source 1..20: mol_type = other RNA
cagggcggtgacggccgtta

SEQ ID NO: 591 - RNA, 20 nt, synthetic construct
  source 1..20: mol_type = other RNA
cctaacggccgtcaccgccc

SEQ ID NO: 592 - RNA, 20 nt, synthetic construct
  source 1..20: mol_type = other RNA
ccgttagggtctgcccccga

SEQ ID NO: 593 - RNA, 20 nt, synthetic construct
  source 1..20: mol_type = other RNA
cgttagggtctgcccccgac

SEQ ID NO: 594 - RNA, 20 nt, synthetic construct
  source 1..20: mol_type = other RNA
ccgtcgggggcagaccctaa

SEQ ID NO: 595 - RNA, 20 nt, synthetic construct
  source 1..20: mol_type = other RNA
gcccccgacgggccaaaaca

SEQ ID NO: 596 - RNA, 20 nt, synthetic construct
  source 1..20: mol_type = other RNA
tccttgttttggcccgtcgg

SEQ ID NO: 597 - RNA, 20 nt, synthetic construct
  source 1..20: mol_type = other RNA
gtccttgttttggcccgtcg

SEQ ID NO: 598 - RNA, 20 nt, synthetic construct
  source 1..20: mol_type = other RNA
tgtccttgttttggcccgtc

SEQ ID NO: 599 - RNA, 20 nt, synthetic construct
  source 1..20: mol_type = other RNA
ttgtccttgttttggcccgt

SEQ ID NO: 600 - RNA, 20 nt, synthetic construct
  source 1..20: mol_type = other RNA
caaaacaaggacaagtggcg

SEQ ID NO: 601 - RNA, 20 nt, synthetic construct
  source 1..20: mol_type = other RNA
ctcgccacttgtccttgttt

SEQ ID NO: 602 - RNA, 20 nt, synthetic construct
  source 1..20: mol_type = other RNA
caaggacaagtggcgaggac

SEQ ID NO: 603 - RNA, 20 nt, synthetic construct
  source 1..20: mol_type = other RNA
aaggacaagtggcgaggact

SEQ ID NO: 604 - RNA, 20 nt, synthetic construct
  source 1..20: mol_type = other RNA
caagtggcgaggactgggcc

SEQ ID NO: 605 - RNA, 20 nt, synthetic construct
  source 1..20: mol_type = other RNA
aagtggcgaggactgggcct

SEQ ID NO: 606 - RNA, 20 nt, synthetic construct
  source 1..20: mol_type = other RNA
agtggcgaggactgggcctg

SEQ ID NO: 607 - RNA, 20 nt, synthetic construct
  source 1..20: mol_type = other RNA
gcgaggactgggcctgggga

SEQ ID NO: 608 - RNA, 20 nt, synthetic construct
  source 1..20: mol_type = other RNA
tgggcctggggatggccctg

SEQ ID NO: 609 - RNA, 20 nt, synthetic construct
  source 1..20: mol_type = other RNA
gggcctggggatggccctgc

SEQ ID NO: 610 - RNA, 20 nt, synthetic construct
  source 1..20: mol_type = other RNA
tggggatggccctgcgggtc

SEQ ID NO: 611 - RNA, 20 nt, synthetic construct
  source 1..20: mol_type = other RNA
ggggatggccctgcgggtcc

SEQ ID NO: 612 - RNA, 20 nt, synthetic construct
  source 1..20: mol_type = other RNA
ggacccgcagggccatcccc

SEQ ID NO: 613 - RNA, 20 nt, synthetic construct
  source 1..20: mol_type = other RNA
tggccctgcgggtccgggcg

SEQ ID NO: 614 - RNA, 20 nt, synthetic construct
  source 1..20: mol_type = other RNA
gcgccgcgcccggacccgca

SEQ ID NO: 615 - RNA, 20 nt, synthetic construct
  source 1..20: mol_type = other RNA
tgcgccgcgcccggacccgc

SEQ ID NO: 616 - RNA, 20 nt, synthetic construct
  source 1..20: mol_type = other RNA
agcaggacttgcgccgcgcc

SEQ ID NO: 617 - RNA, 20 nt, synthetic construct
  source 1..20: mol_type = other RNA
gcaagtcctgctttgtctcc

SEQ ID NO: 618 - RNA, 20 nt, synthetic construct
  source 1..20: mol_type = other RNA
ctgctttgtctccaggtgac

SEQ ID NO: 619 - RNA, 20 nt, synthetic construct
  source 1..20: mol_type = other RNA
cagtcacctggagacaaagc

SEQ ID NO: 620 - RNA, 20 nt, synthetic construct
  source 1..20: mol_type = other RNA
ctccaggtgactggctgtcc

SEQ ID NO: 621 - RNA, 20 nt, synthetic construct
  source 1..20: mol_type = other RNA
aggtgactggctgtccagga

SEQ ID NO: 622 - RNA, 20 nt, synthetic construct
  source 1..20: mol_type = other RNA
tgactggctgtccaggacgg

SEQ ID NO: 623 - RNA, 20 nt, synthetic construct
  source 1..20: mol_type = other RNA
gactggctgtccaggacggc

SEQ ID NO: 624 - RNA, 20 nt, synthetic construct
  source 1..20: mol_type = other RNA
caggacggcgggagctgcta

SEQ ID NO: 625 - RNA, 20 nt, synthetic construct
  source 1..20: mol_type = other RNA
cttagcagctcccgccgtcc

SEQ ID NO: 626 - RNA, 20 nt, synthetic construct
  source 1..20: mol_type = other RNA
gagctgctaaggcttgtgtc

SEQ ID NO: 627 - RNA, 20 nt, synthetic construct
  source 1..20: mol_type = other RNA
tgctaaggcttgtgtccgga

SEQ ID NO: 628 - RNA, 20 nt, synthetic construct
  source 1..20: mol_type = other RNA
cttgtgtccggaaggagcac

SEQ ID NO: 629 - RNA, 20 nt, synthetic construct
  source 1..20: mol_type = other RNA
ttgtgtccggaaggagcaca

SEQ ID NO: 630 - RNA, 20 nt, synthetic construct
  source 1..20: mol_type = other RNA
gtccggaaggagcacaggga

SEQ ID NO: 631 - RNA, 20 nt, synthetic construct
  source 1..20: mol_type = other RNA
tccggaaggagcacagggat

SEQ ID NO: 632 - RNA, 20 nt, synthetic construct
  source 1..20: mol_type = other RNA
gaaggagcacagggatgggc

SEQ ID NO: 633 - RNA, 20 nt, synthetic construct
  source 1..20: mol_type = other RNA
aaggagcacagggatgggca

SEQ ID NO: 634 - RNA, 20 nt, synthetic construct
  source 1..20: mol_type = other RNA
gcccatccctgtgctccttc

SEQ ID NO: 635 - RNA, 20 nt, synthetic construct
  source 1..20: mol_type = other RNA
gagcacagggatgggcaggg

SEQ ID NO: 636 - RNA, 20 nt, synthetic construct
  source 1..20: mol_type = other RNA
acagggatgggcagggtggc

SEQ ID NO: 637 - RNA, 20 nt, synthetic construct
  source 1..20: mol_type = other RNA
cagggatgggcagggtggcc

SEQ ID NO: 638 - RNA, 20 nt, synthetic construct
  source 1..20: mol_type = other RNA
ggcagggtggccgggccagc

SEQ ID NO: 639 - RNA, 20 nt, synthetic construct
  source 1..20: mol_type = other RNA
gatttgagggccggctggcc

SEQ ID NO: 640 - RNA, 20 nt, synthetic construct
  source 1..20: mol_type = other RNA
cggaggatttgagggccggc

SEQ ID NO: 641 - RNA, 20 nt, synthetic construct
  source 1..20: mol_type = other RNA
cctcaaatcctccgacgaag

SEQ ID NO: 642 - RNA, 20 nt, synthetic construct
  source 1..20: mol_type = other RNA
cgcttcgtcggaggatttga

SEQ ID NO: 643 - RNA, 20 nt, synthetic construct
  source 1..20: mol_type = other RNA
ccgcttcgtcggaggatttg

SEQ ID NO: 644 - RNA, 20 nt, synthetic construct
  source 1..20: mol_type = other RNA
ggcggctgccgcttcgtcgg

SEQ ID NO: 645 - RNA, 20 nt, synthetic construct
  source 1..20: mol_type = other RNA
cgtggcggctgccgcttcgt

SEQ ID NO: 646 - RNA, 20 nt, synthetic construct
  source 1..20: mol_type = other RNA
agcggcagccgccacgacca

SEQ ID NO: 647 - RNA, 20 nt, synthetic construct
  source 1..20: mol_type = other RNA
tgctctggccgtggtcgtgg

SEQ ID NO: 648 - RNA, 20 nt, synthetic construct
  source 1..20: mol_type = other RNA
accacggccagagcagcgct

SEQ ID NO: 649 - RNA, 20 nt, synthetic construct
  source 1..20: mol_type = other RNA
acggccagagcagcgctcgg

SEQ ID NO: 650 - RNA, 20 nt, synthetic construct
  source 1..20: mol_type = other RNA
tccgagcgctgctctggccg

SEQ ID NO: 651 - RNA, 20 nt, synthetic construct
  source 1..20: mol_type = other RNA
ctcgcctccgagcgctgctc

SEQ ID NO: 652 - RNA, 20 nt, synthetic construct
  source 1..20: mol_type = other RNA
gtcaacaatcgcctcgcctt

SEQ ID NO: 653 - RNA, 20 nt, synthetic construct
  source 1..20: mol_type = other RNA
aacaatcgcctcgcctttgg

SEQ ID NO: 654 - RNA, 20 nt, synthetic construct
  source 1..20: mol_type = other RNA
gggtcaggccgccaaaggcg

SEQ ID NO: 655 - RNA, 20 nt, synthetic construct
  source 1..20: mol_type = other RNA
cctacgggtcaggccgccaa

SEQ ID NO: 656 - RNA, 20 nt, synthetic construct
  source 1..20: mol_type = other RNA
gggggcggcgcctacgggtc

SEQ ID NO: 657 - RNA, 20 nt, synthetic construct
  source 1..20: mol_type = other RNA
cgtaggcgccgcccccaccg

SEQ ID NO: 658 - RNA, 20 nt, synthetic construct
  source 1..20: mol_type = other RNA
gcggtgggggcggcgcctac

SEQ ID NO: 659 - RNA, 20 nt, synthetic construct
  source 1..20: mol_type = other RNA
cgcggtgggggcggcgccta

SEQ ID NO: 660 - RNA, 20 nt, synthetic construct
  source 1..20: mol_type = other RNA
cccccaccgcggctgccgat

SEQ ID NO: 661 - RNA, 20 nt, synthetic construct
  source 1..20: mol_type = other RNA
atcggcagccgcggtggggg

SEQ ID NO: 662 - RNA, 20 nt, synthetic construct
  source 1..20: mol_type = other RNA
ccaatcggcagccgcggtgg

SEQ ID NO: 663 - RNA, 20 nt, synthetic construct
  source 1..20: mol_type = other RNA
ccgcggctgccgattggctg

SEQ ID NO: 664 - RNA, 20 nt, synthetic construct
  source 1..20: mol_type = other RNA
agccaatcggcagccgcggt

SEQ ID NO: 665 - RNA, 20 nt, synthetic construct
  source 1..20: mol_type = other RNA
cagccaatcggcagccgcgg

SEQ ID NO: 666 - RNA, 20 nt, synthetic construct
  source 1..20: mol_type = other RNA
gctgccgattggctgcggcg

SEQ ID NO: 667 - RNA, 20 nt, synthetic construct
  source 1..20: mol_type = other RNA
cgctccgcgccgcagccaat

SEQ ID NO: 668 - RNA, 20 nt, synthetic construct
  source 1..20: mol_type = other RNA
cggcgcggagcgaccgcgcg

SEQ ID NO: 669 - RNA, 20 nt, synthetic construct
  source 1..20: mol_type = other RNA
gcgaccgcgcgcggaccaat

SEQ ID NO: 670 - RNA, 20 nt, synthetic construct
  source 1..20: mol_type = other RNA
cgaccgcgcgcggaccaatt

SEQ ID NO: 671 - RNA, 20 nt, synthetic construct
  source 1..20: mol_type = other RNA
gcgcggaccaattgggaacg

SEQ ID NO: 672 - RNA, 20 nt, synthetic construct
  source 1..20: mol_type = other RNA
cgcggaccaattgggaacgc

SEQ ID NO: 673 - RNA, 20 nt, synthetic construct
  source 1..20: mol_type = other RNA
caattgggaacgcgggcacc

SEQ ID NO: 674 - RNA, 20 nt, synthetic construct
  source 1..20: mol_type = other RNA
cgggtgcccgcgttcccaat

SEQ ID NO: 675 - RNA, 20 nt, synthetic construct
  source 1..20: mol_type = other RNA
acgcgggcacccggcgccag

SEQ ID NO: 676 - RNA, 20 nt, synthetic construct
  source 1..20: mol_type = other RNA
ggcacccggcgccagcggcg

SEQ ID NO: 677 - RNA, 20 nt, synthetic construct
  source 1..20: mol_type = other RNA
gcacccggcgccagcggcgc

SEQ ID NO: 678 - RNA, 20 nt, synthetic construct
  source 1..20: mol_type = other RNA
cacccggcgccagcggcgcg

SEQ ID NO: 679 - RNA, 20 nt, synthetic construct
  source 1..20: mol_type = other RNA
ccggcgccagcggcgcgggg

SEQ ID NO: 680 - RNA, 20 nt, synthetic construct
  source 1..20: mol_type = other RNA
ctccccgcgccgctggcgcc

SEQ ID NO: 681 - RNA, 20 nt, synthetic construct
  source 1..20: mol_type = other RNA
cctccccgcgccgctggcgc

SEQ ID NO: 682 - RNA, 20 nt, synthetic construct
  source 1..20: mol_type = other RNA
cagcggcgcggggaggtcgg

SEQ ID NO: 683 - RNA, 20 nt, synthetic construct
  source 1..20: mol_type = other RNA
cgccgacctccccgcgccgc

SEQ ID NO: 684 - RNA, 20 nt, synthetic construct
  source 1..20: mol_type = other RNA
cgcggggaggtcggcggtgc

SEQ ID NO: 685 - RNA, 20 nt, synthetic construct
  source 1..20: mol_type = other RNA
ggggaggtcggcggtgccgg

SEQ ID NO: 686 - RNA, 20 nt, synthetic construct
  source 1..20: mol_type = other RNA
gaggtcggcggtgccggcgg

SEQ ID NO: 687 - RNA, 20 nt, synthetic construct
  source 1..20: mol_type = other RNA
gtcggcggtgccggcggcgg

SEQ ID NO: 688 - RNA, 20 nt, synthetic construct
  source 1..20: mol_type = other RNA
tcggcggtgccggcggcggc

SEQ ID NO: 689 - RNA, 20 nt, synthetic construct
  source 1..20: mol_type = other RNA
cgctctgcgcccgccgccgc

SEQ ID NO: 690 - RNA, 20 nt, synthetic construct
  source 1..20: mol_type = other RNA
gcggcgggcgcagagcgcga

SEQ ID NO: 691 - RNA, 20 nt, synthetic construct
  source 1..20: mol_type = other RNA
cggcgggcgcagagcgcgag

SEQ ID NO: 692 - RNA, 20 nt, synthetic construct
  source 1..20: mol_type = other RNA
cgggcgcagagcgcgagggg

SEQ ID NO: 693 - RNA, 20 nt, synthetic construct
  source 1..20: mol_type = other RNA
gcagagcgcgaggggaggag

SEQ ID NO: 694 - RNA, 20 nt, synthetic construct
  source 1..20: mol_type = other RNA
cagagcgcgaggggaggagc

SEQ ID NO: 695 - RNA, 20 nt, synthetic construct
  source 1..20: mol_type = other RNA
agcgcgaggggaggagcggg

SEQ ID NO: 696 - RNA, 20 nt, synthetic construct
  source 1..20: mol_type = other RNA
gcgaggggaggagcgggagg

SEQ ID NO: 697 - RNA, 20 nt, synthetic construct
  source 1..20: mol_type = other RNA
aggggaggagcgggaggagg

SEQ ID NO: 698 - RNA, 20 nt, synthetic construct
  source 1..20: mol_type = other RNA
ggaggagcgggaggaggcgg

SEQ ID NO: 699 - RNA, 20 nt, synthetic construct
  source 1..20: mol_type = other RNA
gaggaggcggaggatgttcc

SEQ ID NO: 700 - RNA, 20 nt, synthetic construct
  source 1..20: mol_type = other RNA
gaggcggaggatgttcccgg

SEQ ID NO: 701 - RNA, 20 nt, synthetic construct
  source 1..20: mol_type = other RNA
gaggatgttcccggcggctg

SEQ ID NO: 702 - RNA, 20 nt, synthetic construct
  source 1..20: mol_type = other RNA
atgttcccggcggctgcggc

SEQ ID NO: 703 - RNA, 20 nt, synthetic construct
  source 1..20: mol_type = other RNA
tgttcccggcggctgcggcc

SEQ ID NO: 704 - RNA, 20 nt, synthetic construct
  source 1..20: mol_type = other RNA
gttcccggcggctgcggccg

SEQ ID NO: 705 - RNA, 20 nt, synthetic construct
  source 1..20: mol_type = other RNA
ctgccccggccgcagccgcc

SEQ ID NO: 706 - RNA, 20 nt, synthetic construct
  source 1..20: mol_type = other RNA
ggctgcggccggggcagcgc

SEQ ID NO: 707 - RNA, 20 nt, synthetic construct
  source 1..20: mol_type = other RNA
gccggggcagcgcgggccag

SEQ ID NO: 708 - RNA, 20 nt, synthetic construct
  source 1..20: mol_type = other RNA
ggcagcgcgggccagaggcg

SEQ ID NO: 709 - RNA, 20 nt, synthetic construct
  source 1..20: mol_type = other RNA
gcctctggcccgcgctgccc

SEQ ID NO: 710 - RNA, 20 nt, synthetic construct
  source 1..20: mol_type = other RNA
cgggccagaggcgcggcgtg

SEQ ID NO: 711 - RNA, 20 nt, synthetic construct
  source 1..20: mol_type = other RNA
ggcgcggcgtgcggagccct

SEQ ID NO: 712 - RNA, 20 nt, synthetic construct
  source 1..20: mol_type = other RNA
gtgcggagccctcggctgcc

SEQ ID NO: 713 - RNA, 20 nt, synthetic construct
  source 1..20: mol_type = other RNA
cggagccctcggctgcccgg

SEQ ID NO: 714 - RNA, 20 nt, synthetic construct
  source 1..20: mol_type = other RNA
ctcggctgcccggcggagcg

SEQ ID NO: 715 - RNA, 20 nt, synthetic construct
  source 1..20: mol_type = other RNA
ggctgcccggcggagcgcgg

SEQ ID NO: 716 - RNA, 20 nt, synthetic construct
  source 1..20: mol_type = other RNA
cgcgctccgccgggcagccg

SEQ ID NO: 717 - RNA, 20 nt, synthetic construct
  source 1..20: mol_type = other RNA
tgcccggcggagcgcggcgg

SEQ ID NO: 718 - RNA, 20 nt, synthetic construct
  source 1..20: mol_type = other RNA
gcccggcggagcgcggcggc

SEQ ID NO: 719 - RNA, 20 nt, synthetic construct
  source 1..20: mol_type = other RNA
ggcggagcgcggcggcgggc

SEQ ID NO: 720 - RNA, 20 nt, synthetic construct
  source 1..20: mol_type = other RNA
gcccgccgccgcgctccgcc

SEQ ID NO: 721 - RNA, 20 nt, synthetic construct
  source 1..20: mol_type = other RNA
agcccgccgccgcgctccgc

SEQ ID NO: 722 - RNA, 20 nt, synthetic construct
  source 1..20: mol_type = other RNA
gagcgcggcggcgggctggc

SEQ ID NO: 723 - RNA, 20 nt, synthetic construct
  source 1..20: mol_type = other RNA
gcggcggcgggctggcggga

SEQ ID NO: 724 - RNA, 20 nt, synthetic construct
  source 1..20: mol_type = other RNA
ggcgggctggcgggaaggcg

SEQ ID NO: 725 - RNA, 20 nt, synthetic construct
  source 1..20: mol_type = other RNA
gcgggctggcgggaaggcgc

SEQ ID NO: 726 - RNA, 20 nt, synthetic construct
  source 1..20: mol_type = other RNA
gcgcgggctttgcgctgcgc

SEQ ID NO: 727 - RNA, 20 nt, synthetic construct
  source 1..20: mol_type = other RNA
cgcgggctttgcgctgcgcc

SEQ ID NO: 728 - RNA, 20 nt, synthetic construct
  source 1..20: mol_type = other RNA
gcgggctttgcgctgcgccg

SEQ ID NO: 729 - RNA, 20 nt, synthetic construct
  source 1..20: mol_type = other RNA
gggactctgaacccgagtcc

SEQ ID NO: 730 - RNA, 20 nt, synthetic construct
  source 1..20: mol_type = other RNA
ggactctgaacccgagtccc

SEQ ID NO: 731 - RNA, 20 nt, synthetic construct
  source 1..20: mol_type = other RNA
ggactcgggttcagagtccc

SEQ ID NO: 732 - RNA, 20 nt, synthetic construct
  source 1..20: mol_type = other RNA
ggagacaaagcccgggactc

SEQ ID NO: 733 - RNA, 20 nt, synthetic construct
  source 1..20: mol_type = other RNA
aggagacaaagcccgggact

SEQ ID NO: 734 - RNA, 20 nt, synthetic construct
  source 1..20: mol_type = other RNA
cagcgcaggagacaaagccc

SEQ ID NO: 735 - RNA, 20 nt, synthetic construct
  source 1..20: mol_type = other RNA
gcagcgcaggagacaaagcc

SEQ ID NO: 736 - RNA, 20 nt, synthetic construct
  source 1..20: mol_type = other RNA
tgtctcctgcgctgctttcg

SEQ ID NO: 737 - RNA, 20 nt, synthetic construct
  source 1..20: mol_type = other RNA
ctgcgctgctttcgtggtga

SEQ ID NO: 738 - RNA, 20 nt, synthetic construct
  source 1..20: mol_type = other RNA
cgtcaccacgaaagcagcgc

SEQ ID NO: 739 - RNA, 20 nt, synthetic construct
  source 1..20: mol_type = other RNA
ctgctttcgtggtgacggtc

SEQ ID NO: 740 - RNA, 20 nt, synthetic construct
  source 1..20: mol_type = other RNA
tgctttcgtggtgacggtca

SEQ ID NO: 741 - RNA, 20 nt, synthetic construct
  source 1..20: mol_type = other RNA
gctttcgtggtgacggtcag

SEQ ID NO: 742 - RNA, 20 nt, synthetic construct
  source 1..20: mol_type = other RNA
ctttcgtggtgacggtcagg

SEQ ID NO: 743 - RNA, 20 nt, synthetic construct
  source 1..20: mol_type = other RNA
ggtgacggtcagggggcgcc

SEQ ID NO: 744 - RNA, 20 nt, synthetic construct
  source 1..20: mol_type = other RNA
acggtcagggggcgcccggt

SEQ ID NO: 745 - RNA, 20 nt, synthetic construct
  source 1..20: mol_type = other RNA
agggggcgcccggtcggcga

SEQ ID NO: 746 - RNA, 20 nt, synthetic construct
  source 1..20: mol_type = other RNA
gggggcgcccggtcggcgaa

SEQ ID NO: 747 - RNA, 20 nt, synthetic construct
  source 1..20: mol_type = other RNA
cgcccggtcggcgaagggcg

SEQ ID NO: 748 - RNA, 20 nt, synthetic construct
  source 1..20: mol_type = other RNA
gcccggtcggcgaagggcgc

SEQ ID NO: 749 - RNA, 20 nt, synthetic construct
  source 1..20: mol_type = other RNA
ggtcggcgaagggcgcgggc

SEQ ID NO: 750 - RNA, 20 nt, synthetic construct
  source 1..20: mol_type = other RNA
gcccgcgcccttcgccgacc

SEQ ID NO: 751 - RNA, 20 nt, synthetic construct
  source 1..20: mol_type = other RNA
ggcccgcgcccttcgccgac

SEQ ID NO: 752 - RNA, 20 nt, synthetic construct
  source 1..20: mol_type = other RNA
agggcgcgggccggacgccg

SEQ ID NO: 753 - RNA, 20 nt, synthetic construct
  source 1..20: mol_type = other RNA
gggcgcgggccggacgccgc

SEQ ID NO: 754 - RNA, 20 nt, synthetic construct
  source 1..20: mol_type = other RNA
ggcgcgggccggacgccgcg

SEQ ID NO: 755 - RNA, 20 nt, synthetic construct
  source 1..20: mol_type = other RNA
gggccggacgccgcggggct

SEQ ID NO: 756 - RNA, 20 nt, synthetic construct
  source 1..20: mol_type = other RNA
acgccgcggggcttggtccc

SEQ ID NO: 757 - RNA, 20 nt, synthetic construct
  source 1..20: mol_type = other RNA
ggaccaagccccgcggcgtc

SEQ ID NO: 758 - RNA, 20 nt, synthetic construct
  source 1..20: mol_type = other RNA
gcggggcttggtccctggcc

SEQ ID NO: 759 - RNA, 20 nt, synthetic construct
  source 1..20: mol_type = other RNA
gggccagggaccaagccccg

SEQ ID NO: 760 - RNA, 20 nt, synthetic construct
  source 1..20: mol_type = other RNA
agagcgcagcgtccgggcca

SEQ ID NO: 761 - RNA, 20 nt, synthetic construct
  source 1..20: mol_type = other RNA
cccggacgctgcgctctgaa

SEQ ID NO: 762 - RNA, 20 nt, synthetic construct
  source 1..20: mol_type = other RNA
gacgctgcgctctgaaggga

SEQ ID NO: 763 - RNA, 20 nt, synthetic construct
  source 1..20: mol_type = other RNA
cccttcagagcgcagcgtcc

SEQ ID NO: 764 - RNA, 20 nt, synthetic construct
  source 1..20: mol_type = other RNA
tcccttcagagcgcagcgtc

SEQ ID NO: 765 - RNA, 20 nt, synthetic construct
  source 1..20: mol_type = other RNA
tgcgctctgaagggaaggcg

SEQ ID NO: 766 - RNA, 20 nt, synthetic construct
  source 1..20: mol_type = other RNA
gaaggcgcggacgtgagttt

SEQ ID NO: 767 - RNA, 20 nt, synthetic construct
  source 1..20: mol_type = other RNA
ttcggtgtgattgccttctg

SEQ ID NO: 768 - RNA, 20 nt, synthetic construct
  source 1..20: mol_type = other RNA
tcggtgtgattgccttctga

SEQ ID NO: 769 - RNA, 20 nt, synthetic construct
  source 1..20: mol_type = other RNA
cggtgtgattgccttctgag

SEQ ID NO: 770 - RNA, 20 nt, synthetic construct
  source 1..20: mol_type = other RNA
tgtgattgccttctgagggg

SEQ ID NO: 771 - RNA, 20 nt, synthetic construct
  source 1..20: mol_type = other RNA
gtgattgccttctgagggga

SEQ ID NO: 772 - RNA, 20 nt, synthetic construct
  source 1..20: mol_type = other RNA
ccttctgaggggagggtctg

SEQ ID NO: 773 - RNA, 20 nt, synthetic construct
  source 1..20: mol_type = other RNA
cttctgaggggagggtctgt

SEQ ID NO: 774 - RNA, 20 nt, synthetic construct
  source 1..20: mol_type = other RNA
ccacagaccctcccctcaga

SEQ ID NO: 775 - RNA, 20 nt, synthetic construct
  source 1..20: mol_type = other RNA
ggggagggtctgtgggatga

SEQ ID NO: 776 - RNA, 20 nt, synthetic construct
  source 1..20: mol_type = other RNA
gagggtctgtgggatgaagg

SEQ ID NO: 777 - RNA, 20 nt, synthetic construct
  source 1..20: mol_type = other RNA
tctgtgggatgaaggcggcg

SEQ ID NO: 778 - RNA, 20 nt, synthetic construct
  source 1..20: mol_type = other RNA
gaaggcggcgcggcgcgcac

SEQ ID NO: 779 - RNA, 20 nt, synthetic construct
  source 1..20: mol_type = other RNA
caccggtgtcgcctagcctg

SEQ ID NO: 780 - RNA, 20 nt, synthetic construct
  source 1..20: mol_type = other RNA
gtccgcaggctaggcgacac

SEQ ID NO: 781 - RNA, 20 nt, synthetic construct
  source 1..20: mol_type = other RNA
tacaactaggtccgcaggct

SEQ ID NO: 782 - RNA, 20 nt, synthetic construct
  source 1..20: mol_type = other RNA
aggtctacaactaggtccgc

SEQ ID NO: 783 - RNA, 20 nt, synthetic construct
  source 1..20: mol_type = other RNA
gacctagttgtagaccttgc

SEQ ID NO: 784 - RNA, 20 nt, synthetic construct
  source 1..20: mol_type = other RNA
cgcctgcaaggtctacaact

SEQ ID NO: 785 - RNA, 20 nt, synthetic construct
  source 1..20: mol_type = other RNA
cgacgaagcgaacgcctgca

SEQ ID NO: 786 - RNA, 20 nt, synthetic construct
  source 1..20: mol_type = other RNA
aatggggagggggcggcgga

SEQ ID NO: 787 - RNA, 20 nt, synthetic construct
  source 1..20: mol_type = other RNA
aaatggggagggggcggcgg

SEQ ID NO: 788 - RNA, 20 nt, synthetic construct
  source 1..20: mol_type = other RNA
tctaaatggggagggggcgg

SEQ ID NO: 789 - RNA, 20 nt, synthetic construct
  source 1..20: mol_type = other RNA
atctctaaatggggaggggg

SEQ ID NO: 790 - RNA, 20 nt, synthetic construct
  source 1..20: mol_type = other RNA
cacatctctaaatggggagg

SEQ ID NO: 791 - RNA, 20 nt, synthetic construct
  source 1..20: mol_type = other RNA
gcacatctctaaatggggag

SEQ ID NO: 792 - RNA, 20 nt, synthetic construct
  source 1..20: mol_type = other RNA
tgcacatctctaaatgggga

SEQ ID NO: 793 - RNA, 20 nt, synthetic construct
  source 1..20: mol_type = other RNA
gtgcacatctctaaatgggg

SEQ ID NO: 794 - RNA, 20 nt, synthetic construct
  source 1..20: mol_type = other RNA
atttagagatgtgcacctca

SEQ ID NO: 795 - RNA, 20 nt, synthetic construct
  source 1..20: mol_type = other RNA
gaggtgcacatctctaaatg

SEQ ID NO: 796 - RNA, 20 nt, synthetic construct
  source 1..20: mol_type = other RNA
tgaggtgcacatctctaaat

SEQ ID NO: 797 - RNA, 20 nt, synthetic construct
  source 1..20: mol_type = other RNA
gtgaggtgcacatctctaaa

SEQ ID NO: 798 - RNA, 20 nt, synthetic construct
  source 1..20: mol_type = other RNA
tctctgaggtgcacaccgtg

SEQ ID NO: 799 - RNA, 20 nt, synthetic construct
  source 1..20: mol_type = other RNA
cagagaagttctgtctgatt

SEQ ID NO: 800 - RNA, 20 nt, synthetic construct
  source 1..20: mol_type = other RNA
aatcagacagaacttctctg

SEQ ID NO: 801 - RNA, 20 nt, synthetic construct
  source 1..20: mol_type = other RNA
aagttctgtctgattcggtg

SEQ ID NO: 802 - RNA, 20 nt, synthetic construct
  source 1..20: mol_type = other RNA
gtctgattcggtgcggcgtg

SEQ ID NO: 803 - RNA, 20 nt, synthetic construct
  source 1..20: mol_type = other RNA
attcggtgcggcgtgcggta

SEQ ID NO: 804 - RNA, 20 nt, synthetic construct
  source 1..20: mol_type = other RNA
ttcggtgcggcgtgcggtac

SEQ ID NO: 805 - RNA, 20 nt, synthetic construct
  source 1..20: mol_type = other RNA
tgcggcgtgcggtacgggag

SEQ ID NO: 806 - RNA, 20 nt, synthetic construct
  source 1..20: mol_type = other RNA
gcggcgtgcggtacgggagc

SEQ ID NO: 807 - RNA, 20 nt, synthetic construct
  source 1..20: mol_type = other RNA
gcgtgcggtacgggagcggg

SEQ ID NO: 808 - RNA, 20 nt, synthetic construct
  source 1..20: mol_type = other RNA
cgtgcggtacgggagcggga

SEQ ID NO: 809 - RNA, 20 nt, synthetic construct
  source 1..20: mol_type = other RNA
gcggtacgggagcgggaggg

SEQ ID NO: 810 - RNA, 20 nt, synthetic construct
  source 1..20: mol_type = other RNA
cggtacgggagcgggaggga

SEQ ID NO: 811 - RNA, 20 nt, synthetic construct
  source 1..20: mol_type = other RNA
ggagcgggagggagggagca

SEQ ID NO: 812 - RNA, 20 nt, synthetic construct
  source 1..20: mol_type = other RNA
gagcgggagggagggagcac

SEQ ID NO: 813 - RNA, 20 nt, synthetic construct
  source 1..20: mol_type = other RNA
cgggagggagggagcacggg

SEQ ID NO: 814 - RNA, 20 nt, synthetic construct
  source 1..20: mol_type = other RNA
ggcggagagagcgccagagc

SEQ ID NO: 815 - RNA, 20 nt, synthetic construct
  source 1..20: mol_type = other RNA
gcggagagagcgccagagcc

SEQ ID NO: 816 - RNA, 20 nt, synthetic construct
  source 1..20: mol_type = other RNA
agagccgggccgagccgcgc

SEQ ID NO: 817 - RNA, 20 nt, synthetic construct
  source 1..20: mol_type = other RNA
agcgcggctcggcccggctc

SEQ ID NO: 818 - RNA, 20 nt, synthetic construct
  source 1..20: mol_type = other RNA
aactccagcgcggctcggcc

SEQ ID NO: 819 - RNA, 20 nt, synthetic construct
  source 1..20: mol_type = other RNA
tttgtaactccagcgcggct

SEQ ID NO: 820 - RNA, 20 nt, synthetic construct
  source 1..20: mol_type = other RNA
tagagtttgtaactccagcg

SEQ ID NO: 821 - RNA, 20 nt, synthetic construct
  source 1..20: mol_type = other RNA
gacgcacttactacgactga

SEQ ID NO: 822 - RNA, 20 nt, synthetic construct
  source 1..20: mol_type = other RNA
gtctggggaaggtctggcag

SEQ ID NO: 823 - RNA, 20 nt, synthetic construct
  source 1..20: mol_type = other RNA
cagcaagtctggggaaggtc

SEQ ID NO: 824 - RNA, 20 nt, synthetic construct
  source 1..20: mol_type = other RNA
gagggcagcaagtctgggga

SEQ ID NO: 825 - RNA, 20 nt, synthetic construct
  source 1..20: mol_type = other RNA
tgctgagggcagcaagtctg

SEQ ID NO: 826 - RNA, 20 nt, synthetic construct
  source 1..20: mol_type = other RNA
atgctgagggcagcaagtct

SEQ ID NO: 827 - RNA, 20 nt, synthetic construct
  source 1..20: mol_type = other RNA
cttgctgccctcagcatttt

SEQ ID NO: 828 - RNA, 20 nt, synthetic construct
  source 1..20: mol_type = other RNA
tcagcattttcggcaaacaa

SEQ ID NO: 829 - RNA, 20 nt, synthetic construct
  source 1..20: mol_type = other RNA
cagcattttcggcaaacaat

SEQ ID NO: 830 - RNA, 20 nt, synthetic construct
  source 1..20: mol_type = other RNA
agcattttcggcaaacaatg

SEQ ID NO: 831 - RNA, 20 nt, synthetic construct
  source 1..20: mol_type = other RNA
attgtttgccgaaaatgctg

SEQ ID NO: 832 - RNA, 20 nt, synthetic construct
  source 1..20: mol_type = other RNA
ttttcggcaaacaatggggc

SEQ ID NO: 833 - RNA, 20 nt, synthetic construct
  source 1..20: mol_type = other RNA
gcaaacaatggggccggagc

SEQ ID NO: 834 - RNA, 20 nt, synthetic construct
  source 1..20: mol_type = other RNA
caaacaatggggccggagca

SEQ ID NO: 835 - RNA, 20 nt, synthetic construct
  source 1..20: mol_type = other RNA
tggggccggagcagggaacg

SEQ ID NO: 836 - RNA, 20 nt, synthetic construct
  source 1..20: mol_type = other RNA
gctggccgcgttccctgctc

SEQ ID NO: 837 - RNA, 20 nt, synthetic construct
  source 1..20: mol_type = other RNA
atgcagcgattgcaggcggc

SEQ ID NO: 838 - RNA, 20 nt, synthetic construct
  source 1..20: mol_type = other RNA
gcagatgcagcgattgcagg

SEQ ID NO: 839 - RNA, 20 nt, synthetic construct
  source 1..20: mol_type = other RNA
ggcgcagatgcagcgattgc

SEQ ID NO: 840 - RNA, 20 nt, synthetic construct
  source 1..20: mol_type = other RNA
ctgcgcccgctcctgtgctc

SEQ ID NO: 841 - RNA, 20 nt, synthetic construct
  source 1..20: mol_type = other RNA
ggacgccggagcacaggagc

SEQ ID NO: 842 - RNA, 20 nt, synthetic construct
  source 1..20: mol_type = other RNA
aggacgccggagcacaggag

SEQ ID NO: 843 - RNA, 20 nt, synthetic construct
  source 1..20: mol_type = other RNA
taggtaggacgccggagcac

SEQ ID NO: 844 - RNA, 20 nt, synthetic construct
  source 1..20: mol_type = other RNA
tccggcgtcctacctaaccc

SEQ ID NO: 845 - RNA, 20 nt, synthetic construct
  source 1..20: mol_type = other RNA
ccggcgtcctacctaacccc

SEQ ID NO: 846 - RNA, 20 nt, synthetic construct
  source 1..20: mol_type = other RNA
cccggggttaggtaggacgc

SEQ ID NO: 847 - RNA, 20 nt, synthetic construct
  source 1..20: mol_type = other RNA
ctgacttcccggggttaggt

SEQ ID NO: 848 - RNA, 20 nt, synthetic construct
  source 1..20: mol_type = other RNA
ggctctgacttcccggggtt

SEQ ID NO: 849 - RNA, 20 nt, synthetic construct
  source 1..20: mol_type = other RNA
cccgggaagtcagagccgct

SEQ ID NO: 850 - RNA, 20 nt, synthetic construct
  source 1..20: mol_type = other RNA
ccagcggctctgacttcccg

SEQ ID NO: 851 - RNA, 20 nt, synthetic construct
  source 1..20: mol_type = other RNA
cccagcggctctgacttccc

SEQ ID NO: 852 - RNA, 20 nt, synthetic construct
  source 1..20: mol_type = other RNA
tcccagcggctctgacttcc

SEQ ID NO: 853 - RNA, 20 nt, synthetic construct
  source 1..20: mol_type = other RNA
agtaagtcagaaactcccag

SEQ ID NO: 854 - RNA, 20 nt, synthetic construct
  source 1..20: mol_type = other RNA
ttactcgaagaagtctgtcc

SEQ ID NO: 855 - RNA, 20 nt, synthetic construct
  source 1..20: mol_type = other RNA
tactcgaagaagtctgtcct

SEQ ID NO: 856 - RNA, 20 nt, synthetic construct
  source 1..20: mol_type = other RNA
ttcgtgtgtgctctttgccc

SEQ ID NO: 857 - RNA, 20 nt, synthetic construct
  source 1..20: mol_type = other RNA
cttcagattagctgcttctc

SEQ ID NO: 858 - RNA, 20 nt, synthetic construct
  source 1..20: mol_type = other RNA
atgtcaacagcttgcggaac

SEQ ID NO: 859 - RNA, 20 nt, synthetic construct
  source 1..20: mol_type = other RNA
gtaacaatgtcaacagcttg

SEQ ID NO: 860 - RNA, 20 nt, synthetic construct
  source 1..20: mol_type = other RNA
cattgttactgtattttgtt

SEQ ID NO: 861 - RNA, 20 nt, synthetic construct
  source 1..20: mol_type = other RNA
attgttactgtattttgttt

SEQ ID NO: 862 - RNA, 20 nt, synthetic construct
  source 1..20: mol_type = other RNA
ttgttactgtattttgtttg

SEQ ID NO: 863 - RNA, 20 nt, synthetic construct
  source 1..20: mol_type = other RNA
tgttactgtattttgtttgg

SEQ ID NO: 864 - RNA, 20 nt, synthetic construct
  source 1..20: mol_type = other RNA
tgtaatttttttttggtaga

SEQ ID NO: 865 - RNA, 20 nt, synthetic construct
  source 1..20: mol_type = other RNA
gtgtaatttttttttggtag

SEQ ID NO: 866 - RNA, 20 nt, synthetic construct
  source 1..20: mol_type = other RNA
ataaaggtgtaatttttttt

SEQ ID NO: 867 - RNA, 20 nt, synthetic construct
  source 1..20: mol_type = other RNA
aattacacctttattatttt

SEQ ID NO: 868 - RNA, 20 nt, synthetic construct
  source 1..20: mol_type = other RNA
aattgcacctaaaataataa

SEQ ID NO: 869 - RNA, 20 nt, synthetic construct
  source 1..20: mol_type = other RNA
ttaggtgcaatttttttatt

SEQ ID NO: 870 - RNA, 20 nt, synthetic construct
  source 1..20: mol_type = other RNA
taggtgcaatttttttattt

SEQ ID NO: 871 - RNA, 20 nt, synthetic construct
  source 1..20: mol_type = other RNA
cctaagaatttttaatcgct

SEQ ID NO: 872 - RNA, 20 nt, synthetic construct
  source 1..20: mol_type = other RNA
ctagcgattaaaaattctta

SEQ ID NO: 873 - RNA, 20 nt, synthetic construct
  source 1..20: mol_type = other RNA
cctagcgattaaaaattctt

SEQ ID NO: 874 - RNA, 20 nt, synthetic construct
  source 1..20: mol_type = other RNA
ttgcagaaaaaaagaccaaa

SEQ ID NO: 875 - RNA, 20 nt, synthetic construct
  source 1..20: mol_type = other RNA
ctgcccccacggcagccctc

SEQ ID NO: 876 - RNA, 20 nt, synthetic construct
  source 1..20: mol_type = other RNA
tgcccccacggcagccctca

SEQ ID NO: 877 - RNA, 20 nt, synthetic construct
  source 1..20: mol_type = other RNA
ggccctgagggctgccgtgg

SEQ ID NO: 878 - RNA, 20 nt, synthetic construct
  source 1..20: mol_type = other RNA
gggccctgagggctgccgtg

SEQ ID NO: 879 - RNA, 20 nt, synthetic construct
  source 1..20: mol_type = other RNA
cgggccctgagggctgccgt

SEQ ID NO: 880 - RNA, 20 nt, synthetic construct
  source 1..20: mol_type = other RNA
gcgggccctgagggctgccg

SEQ ID NO: 881 - RNA, 20 nt, synthetic construct
  source 1..20: mol_type = other RNA
gtggggccagcgggccctga

SEQ ID NO: 882 - RNA, 20 nt, synthetic construct
  source 1..20: mol_type = other RNA
ggtggggccagcgggccctg

SEQ ID NO: 883 - RNA, 20 nt, synthetic construct
  source 1..20: mol_type = other RNA
ctggccccacctgccagccc

SEQ ID NO: 884 - RNA, 20 nt, synthetic construct
  source 1..20: mol_type = other RNA
ggctggcaggtggggccagc

SEQ ID NO: 885 - RNA, 20 nt, synthetic construct
  source 1..20: mol_type = other RNA
gggctggcaggtggggccag

SEQ ID NO: 886 - RNA, 20 nt, synthetic construct
  source 1..20: mol_type = other RNA
agggccagggctggcaggtg

SEQ ID NO: 887 - RNA, 20 nt, synthetic construct
  source 1..20: mol_type = other RNA
aagggccagggctggcaggt

SEQ ID NO: 888 - RNA, 20 nt, synthetic construct
  source 1..20: mol_type = other RNA
aaagggccagggctggcagg

SEQ ID NO: 889 - RNA, 20 nt, synthetic construct
  source 1..20: mol_type = other RNA
gcaaaagggccagggctggc

SEQ ID NO: 890 - RNA, 20 nt, synthetic construct
  source 1..20: mol_type = other RNA
ggtagcaaaagggccagggc

SEQ ID NO: 891 - RNA, 20 nt, synthetic construct
  source 1..20: mol_type = other RNA
atctggtagcaaaagggcca

SEQ ID NO: 892 - RNA, 20 nt, synthetic construct
  source 1..20: mol_type = other RNA
gatctggtagcaaaagggcc

SEQ ID NO: 893 - RNA, 20 nt, synthetic construct
  source 1..20: mol_type = other RNA
gcggggatctggtagcaaaa

SEQ ID NO: 894 - RNA, 20 nt, synthetic construct
  source 1..20: mol_type = other RNA
agcggggatctggtagcaaa

SEQ ID NO: 895 - RNA, 20 nt, synthetic construct
  source 1..20: mol_type = other RNA
aaagatgaaaagcggggatc

SEQ ID NO: 896 - RNA, 20 nt, synthetic construct
  source 1..20: mol_type = other RNA
tctcataaagatgaaaagcg

SEQ ID NO: 897 - RNA, 20 nt, synthetic construct
  source 1..20: mol_type = other RNA
ttctcataaagatgaaaagc

SEQ ID NO: 898 - RNA, 20 nt, synthetic construct
  source 1..20: mol_type = other RNA
cttctcataaagatgaaaag

SEQ ID NO: 899 - RNA, 20 nt, synthetic construct
  source 1..20: mol_type = other RNA
tgcaatgggtaagcaatgcc

SEQ ID NO: 900 - RNA, 20 nt, synthetic construct
  source 1..20: mol_type = other RNA
gcaatgggtaagcaatgcct

SEQ ID NO: 901 - RNA, 20 nt, synthetic construct
  source 1..20: mol_type = other RNA
gtaagcaatgcctgggtaag

SEQ ID NO: 902 - RNA, 20 nt, synthetic construct
  source 1..20: mol_type = other RNA
ggtaagaggcagttgacgtg

SEQ ID NO: 903 - RNA, 20 nt, synthetic construct
  source 1..20: mol_type = other RNA
acgtcaactgcctcttaccc

SEQ ID NO: 904 - RNA, 20 nt, synthetic construct
  source 1..20: mol_type = other RNA
agaggcagttgacgtgtgga

SEQ ID NO: 905 - RNA, 20 nt, synthetic construct
  source 1..20: mol_type = other RNA
ggatggttgaatctgcttga

SEQ ID NO: 906 - RNA, 20 nt, synthetic construct
  source 1..20: mol_type = other RNA
atctgcttgaaggctgtgtg

SEQ ID NO: 907 - RNA, 20 nt, synthetic construct
  source 1..20: mol_type = other RNA
cagttacggggttttaaaag

SEQ ID NO: 908 - RNA, 20 nt, synthetic construct
  source 1..20: mol_type = other RNA
tcagttacggggttttaaaa

SEQ ID NO: 909 - RNA, 20 nt, synthetic construct
  source 1..20: mol_type = other RNA
atcagttacggggttttaaa

SEQ ID NO: 910 - RNA, 20 nt, synthetic construct
  source 1..20: mol_type = other RNA
gatggaataaatcagttacg

SEQ ID NO: 911 - RNA, 20 nt, synthetic construct
  source 1..20: mol_type = other RNA
agatggaataaatcagttac

SEQ ID NO: 912 - RNA, 20 nt, synthetic construct
  source 1..20: mol_type = other RNA
aagatggaataaatcagtta

SEQ ID NO: 913 - RNA, 20 nt, synthetic construct
  source 1..20: mol_type = other RNA
tgatttattccatctttaga

SEQ ID NO: 914 - RNA, 20 nt, synthetic construct
  source 1..20: mol_type = other RNA
gatttattccatctttagat

SEQ ID NO: 915 - RNA, 20 nt, synthetic construct
  source 1..20: mol_type = other RNA
catcatgctgttctccatag

SEQ ID NO: 916 - RNA, 20 nt, synthetic construct
  source 1..20: mol_type = other RNA
ctctatggagaacagcatga

SEQ ID NO: 917 - RNA, 20 nt, synthetic construct
  source 1..20: mol_type = other RNA
gtaaaatggcacagcctcta

SEQ ID NO: 918 - RNA, 20 nt, synthetic construct
  source 1..20: mol_type = other RNA
cattttacattcccaccaac

SEQ ID NO: 919 - RNA, 20 nt, synthetic construct
  source 1..20: mol_type = other RNA
attttacattcccaccaaca

SEQ ID NO: 920 - RNA, 20 nt, synthetic construct
  source 1..20: mol_type = other RNA
ctgttggtgggaatgtaaaa

SEQ ID NO: 921 - RNA, 20 nt, synthetic construct
  source 1..20: mol_type = other RNA
attcccaccaacagggcaca

SEQ ID NO: 922 - RNA, 20 nt, synthetic construct
  source 1..20: mol_type = other RNA
ttcccaccaacagggcacaa

SEQ ID NO: 923 - RNA, 20 nt, synthetic construct
  source 1..20: mol_type = other RNA
aacccttgtgccctgttggt

SEQ ID NO: 924 - RNA, 20 nt, synthetic construct
  source 1..20: mol_type = other RNA
gaacccttgtgccctgttgg

SEQ ID NO: 925 - RNA, 20 nt, synthetic construct
  source 1..20: mol_type = other RNA
ctggaacccttgtgccctgt

SEQ ID NO: 926 - RNA, 20 nt, synthetic construct
  source 1..20: mol_type = other RNA
tggtaagtatgtggagaaac

SEQ ID NO: 927 - RNA, 20 nt, synthetic construct
  source 1..20: mol_type = other RNA
aaaaagtgttggtaagtatg

SEQ ID NO: 928 - RNA, 20 nt, synthetic construct
  source 1..20: mol_type = other RNA
aaaaaaaaaaaaaaaagtgt

SEQ ID NO: 929 - RNA, 20 nt, synthetic construct
  source 1..20: mol_type = other RNA
tgctttggatttatatttac

SEQ ID NO: 930 - RNA, 20 nt, synthetic construct
  source 1..20: mol_type = other RNA
tttactggcttagatttgta

SEQ ID NO: 931 - RNA, 20 nt, synthetic construct
  source 1..20: mol_type = other RNA
ctgtatcttgactatggtgg

SEQ ID NO: 932 - RNA, 20 nt, synthetic construct
  source 1..20: mol_type = other RNA
gttctgtatcttgactatgg

SEQ ID NO: 933 - RNA, 20 nt, synthetic construct
  source 1..20: mol_type = other RNA
gttgttctgtatcttgacta

SEQ ID NO: 934 - RNA, 20 nt, synthetic construct
  source 1..20: mol_type = other RNA
tacagaacaactcaaccaca

SEQ ID NO: 935 - RNA, 20 nt, synthetic construct
  source 1..20: mol_type = other RNA
ggtatcatgagaaatccttg

SEQ ID NO: 936 - RNA, 20 nt, synthetic construct
  source 1..20: mol_type = other RNA
aggtggctgtggctataaaa

SEQ ID NO: 937 - RNA, 20 nt, synthetic construct
  source 1..20: mol_type = other RNA
aagagggagagaggtggctg

SEQ ID NO: 938 - RNA, 20 nt, synthetic construct
  source 1..20: mol_type = other RNA
tcaaggaagagggagagagg

SEQ ID NO: 939 - RNA, 20 nt, synthetic construct
  source 1..20: mol_type = other RNA
tgctcaaggaagagggagag

SEQ ID NO: 940 - RNA, 20 nt, synthetic construct
  source 1..20: mol_type = other RNA
gacaaaatgctcaaggaaga

SEQ ID NO: 941 - RNA, 20 nt, synthetic construct
  source 1..20: mol_type = other RNA
tccttgagcattttgtcata

SEQ ID NO: 942 - RNA, 20 nt, synthetic construct
  source 1..20: mol_type = other RNA
accatatgacaaaatgctca

SEQ ID NO: 943 - RNA, 20 nt, synthetic construct
  source 1..20: mol_type = other RNA
gcattttgtcatatggtcat

SEQ ID NO: 944 - RNA, 20 nt, synthetic construct
  source 1..20: mol_type = other RNA
caaacacagtgtccttcaac

SEQ ID NO: 945 - RNA, 20 nt, synthetic construct
  source 1..20: mol_type = other RNA
gacactgtgtttgcatgttc

SEQ ID NO: 946 - RNA, 20 nt, synthetic construct
  source 1..20: mol_type = other RNA
tgtgtttgcatgttctggca

SEQ ID NO: 947 - RNA, 20 nt, synthetic construct
  source 1..20: mol_type = other RNA
tgcatgttctggcaaggccc

SEQ ID NO: 948 - RNA, 20 nt, synthetic construct
  source 1..20: mol_type = other RNA
tggcaaggccctggcacagc

SEQ ID NO: 949 - RNA, 20 nt, synthetic construct
  source 1..20: mol_type = other RNA
ccctggcacagctggaactc

SEQ ID NO: 950 - RNA, 20 nt, synthetic construct
  source 1..20: mol_type = other RNA
cctggcacagctggaactca

SEQ ID NO: 951 - RNA, 20 nt, synthetic construct
  source 1..20: mol_type = other RNA
ggcacagctggaactcaggg

SEQ ID NO: 952 - RNA, 20 nt, synthetic construct
  source 1..20: mol_type = other RNA
cctgagttccagctgtgcca

SEQ ID NO: 953 - RNA, 20 nt, synthetic construct
  source 1..20: mol_type = other RNA
ccctgagttccagctgtgcc

SEQ ID NO: 954 - RNA, 20 nt, synthetic construct
  source 1..20: mol_type = other RNA
ggagtgcactggtgcgatct

SEQ ID NO: 955 - RNA, 20 nt, synthetic construct
  source 1..20: mol_type = other RNA
ctccaactcccaagttcaag

SEQ ID NO: 956 - RNA, 20 nt, synthetic construct
  source 1..20: mol_type = other RNA
cgcttgaacttgggagttgg

SEQ ID NO: 957 - RNA, 20 nt, synthetic construct
  source 1..20: mol_type = other RNA
aaccgcttgaacttgggagt

SEQ ID NO: 958 - RNA, 20 nt, synthetic construct
  source 1..20: mol_type = other RNA
caggagaaccgcttgaactt

SEQ ID NO: 959 - RNA, 20 nt, synthetic construct
  source 1..20: mol_type = other RNA
gcaggagaaccgcttgaact

SEQ ID NO: 960 - RNA, 20 nt, synthetic construct
  source 1..20: mol_type = other RNA
gcctcagcctcccaagtagc

SEQ ID NO: 961 - RNA, 20 nt, synthetic construct
  source 1..20: mol_type = other RNA
cctcagcctcccaagtagct

SEQ ID NO: 962 - RNA, 20 nt, synthetic construct
  source 1..20: mol_type = other RNA
gctacttgggaggctgaggc

SEQ ID NO: 963 - RNA, 20 nt, synthetic construct
  source 1..20: mol_type = other RNA
cccagctacttgggaggctg

SEQ ID NO: 964 - RNA, 20 nt, synthetic construct
  source 1..20: mol_type = other RNA
tcccaagtagctgggattac

SEQ ID NO: 965 - RNA, 20 nt, synthetic construct
  source 1..20: mol_type = other RNA
tgtaatcccagctacttggg

SEQ ID NO: 966 - RNA, 20 nt, synthetic construct
  source 1..20: mol_type = other RNA
gcctgtaatcccagctactt

SEQ ID NO: 967 - RNA, 20 nt, synthetic construct
  source 1..20: mol_type = other RNA
tgcctgtaatcccagctact

SEQ ID NO: 968 - RNA, 20 nt, synthetic construct
  source 1..20: mol_type = other RNA
caaaaattagctgggtgtgg

SEQ ID NO: 969 - RNA, 20 nt, synthetic construct
  source 1..20: mol_type = other RNA
atacaaaaattagctgggtg

SEQ ID NO: 970 - RNA, 20 nt, synthetic construct
  source 1..20: mol_type = other RNA
taaaaatacaaaaattagct

SEQ ID NO: 971 - RNA, 20 nt, synthetic construct
  source 1..20: mol_type = other RNA
ataaaaatacaaaaattagc

SEQ ID NO: 972 - RNA, 20 nt, synthetic construct
  source 1..20: mol_type = other RNA
ttttgtatttttattagaga

SEQ ID NO: 973 - RNA, 20 nt, synthetic construct
  source 1..20: mol_type = other RNA
tttgtatttttattagagat

SEQ ID NO: 974 - RNA, 20 nt, synthetic construct
  source 1..20: mol_type = other RNA
agagatgggtttcaccatgt

SEQ ID NO: 975 - RNA, 20 nt, synthetic construct
  source 1..20: mol_type = other RNA
tgggtttcaccatgttggcc

SEQ ID NO: 976 - RNA, 20 nt, synthetic construct
  source 1..20: mol_type = other RNA
tttcaccatgttggccaggc

SEQ ID NO: 977 - RNA, 20 nt, synthetic construct
  source 1..20: mol_type = other RNA
cgagaccagcctggccaaca

SEQ ID NO: 978 - RNA, 20 nt, synthetic construct
  source 1..20: mol_type = other RNA
tcaggagttcgagaccagcc

SEQ ID NO: 979 - RNA, 20 nt, synthetic construct
  source 1..20: mol_type = other RNA
ggtctcgaactcctgacctc

SEQ ID NO: 980 - RNA, 20 nt, synthetic construct
  source 1..20: mol_type = other RNA
cgggcagatcacctgaggtc

SEQ ID NO: 981 - RNA, 20 nt, synthetic construct
  source 1..20: mol_type = other RNA
ctcaggtgatctgcccgcct

SEQ ID NO: 982 - RNA, 20 nt, synthetic construct
  source 1..20: mol_type = other RNA
caaggcgggcagatcacctg

SEQ ID NO: 983 - RNA, 20 nt, synthetic construct
  source 1..20: mol_type = other RNA
gccttggcctcccaaagtgt

SEQ ID NO: 984 - RNA, 20 nt, synthetic construct
  source 1..20: mol_type = other RNA
ccttggcctcccaaagtgtt

SEQ ID NO: 985 - RNA, 20 nt, synthetic construct
  source 1..20: mol_type = other RNA
attagcacaagtgcaagtta

SEQ ID NO: 986 - RNA, 20 nt, synthetic construct
  source 1..20: mol_type = other RNA
cacagaaggaaaagaacagg

SEQ ID NO: 987 - RNA, 20 nt, synthetic construct
  source 1..20: mol_type = other RNA
tgtcacagaaggaaaagaac

SEQ ID NO: 988 - RNA, 20 nt, synthetic construct
  source 1..20: mol_type = other RNA
ataacttgttttgtcacaga

SEQ ID NO: 989 - RNA, 20 nt, synthetic construct
  source 1..20: mol_type = other RNA
gacaaaacaagttatctgtc

SEQ ID NO: 990 - RNA, 20 nt, synthetic construct
  source 1..20: mol_type = other RNA
acaaaacaagttatctgtct

SEQ ID NO: 991 - RNA, 20 nt, synthetic construct
  source 1..20: mol_type = other RNA
gttatctgtctgggaagaca

SEQ ID NO: 992 - RNA, 20 nt, synthetic construct
  source 1..20: mol_type = other RNA
gattttgctaaccacttgag

SEQ ID NO: 993 - RNA, 20 nt, synthetic construct
  source 1..20: mol_type = other RNA
gtttttctttttattcaaaa

SEQ ID NO: 994 - RNA, 20 nt, synthetic construct
  source 1..20: mol_type = other RNA
tttttctttttattcaaaat

SEQ ID NO: 995 - RNA, 20 nt, synthetic construct
  source 1..20: mol_type = other RNA
tctcacttaaaagtcacaaa

SEQ ID NO: 996 - RNA, 20 nt, synthetic construct
  source 1..20: mol_type = other RNA
attattgataacacactgta

SEQ ID NO: 997 - RNA, 20 nt, synthetic construct
  source 1..20: mol_type = other RNA
gattattgataacacactgt

SEQ ID NO: 998 - RNA, 20 nt, synthetic construct
  source 1..20: mol_type = other RNA
tctgagaaccgtcagagttg

SEQ ID NO: 999 - RNA, 20 nt, synthetic construct
  source 1..20: mol_type = other RNA
tttgaaatcctcaactctga

SEQ ID NO: 1000 - RNA, 20 nt, synthetic construct
  source 1..20: mol_type = other RNA
gcatttaccgcaaacgctga

SEQ ID NO: 1001 - RNA, 20 nt, synthetic construct
  source 1..20: mol_type = other RNA
gcaactgccatcagcgtttg

SEQ ID NO: 1002 - RNA, 20 nt, synthetic construct
  source 1..20: mol_type = other RNA
tcctttgccttatagctaac

SEQ ID NO: 1003 - RNA, 20 nt, synthetic construct
  source 1..20: mol_type = other RNA
cctttgccttatagctaact

SEQ ID NO: 1004 - RNA, 20 nt, synthetic construct
  source 1..20: mol_type = other RNA
cccagttagctataaggcaa

SEQ ID NO: 1005 - RNA, 20 nt, synthetic construct
  source 1..20: mol_type = other RNA
tctagtcccagttagctata

SEQ ID NO: 1006 - RNA, 20 nt, synthetic construct
  source 1..20: mol_type = other RNA
tagaaacagctccatcaccc

SEQ ID NO: 1007 - RNA, 20 nt, synthetic construct
  source 1..20: mol_type = other RNA
tcacccaggtgagttttata

SEQ ID NO: 1008 - RNA, 20 nt, synthetic construct
  source 1..20: mol_type = other RNA
tataaaactcacctgggtga

SEQ ID NO: 1009 - RNA, 20 nt, synthetic construct
  source 1..20: mol_type = other RNA
tttccttataaaactcacct

SEQ ID NO: 1010 - RNA, 20 nt, synthetic construct
  source 1..20: mol_type = other RNA
gtttccttataaaactcacc

SEQ ID NO: 1011 - RNA, 20 nt, synthetic construct
  source 1..20: mol_type = other RNA
gagttttataaggaaacata

SEQ ID NO: 1012 - RNA, 20 nt, synthetic construct
  source 1..20: mol_type = other RNA
agttttataaggaaacataa

SEQ ID NO: 1013 - RNA, 20 nt, synthetic construct
  source 1..20: mol_type = other RNA
gttttataaggaaacataag

SEQ ID NO: 1014 - RNA, 20 nt, synthetic construct
  source 1..20: mol_type = other RNA
ttttataaggaaacataagg

SEQ ID NO: 1015 - RNA, 20 nt, synthetic construct
  source 1..20: mol_type = other RNA
ataaggaaacataagggggc

SEQ ID NO: 1016 - RNA, 20 nt, synthetic construct
  source 1..20: mol_type = other RNA
ttccctcctcttgtaagctt

SEQ ID NO: 1017 - RNA, 20 nt, synthetic construct
  source 1..20: mol_type = other RNA
atccaaagcttacaagagga

SEQ ID NO: 1018 - RNA, 20 nt, synthetic construct
  source 1..20: mol_type = other RNA
tatccaaagcttacaagagg

SEQ ID NO: 1019 - RNA, 20 nt, synthetic construct
  source 1..20: mol_type = other RNA
agttatccaaagcttacaag

SEQ ID NO: 1020 - RNA, 20 nt, synthetic construct
  source 1..20: mol_type = other RNA
tttctgaagatatttaaaga

SEQ ID NO: 1021 - RNA, 20 nt, synthetic construct
  source 1..20: mol_type = other RNA
taagaagtttgaagattcag

SEQ ID NO: 1022 - RNA, 20 nt, synthetic construct
  source 1..20: mol_type = other RNA
agattcagtggacacacttt

SEQ ID NO: 1023 - RNA, 20 nt, synthetic construct
  source 1..20: mol_type = other RNA
attataaaagttttgattag

SEQ ID NO: 1024 - RNA, 20 nt, synthetic construct
  source 1..20: mol_type = other RNA
aagtaaagagaaagaaaaca

SEQ ID NO: 1025 - RNA, 20 nt, synthetic construct
  source 1..20: mol_type = other RNA
aagaaaacatggatctgcct

SEQ ID NO: 1026 - RNA, 20 nt, synthetic construct
  source 1..20: mol_type = other RNA
tcaggcagaggtgacttcct

SEQ ID NO: 1027 - RNA, 20 nt, synthetic construct
  source 1..20: mol_type = other RNA
tgcctgagtctgctacttgc

SEQ ID NO: 1028 - RNA, 20 nt, synthetic construct
  source 1..20: mol_type = other RNA
caagtagcagactcaggcag

SEQ ID NO: 1029 - RNA, 20 nt, synthetic construct
  source 1..20: mol_type = other RNA
gagtctgctacttgcaggat

SEQ ID NO: 1030 - RNA, 20 nt, synthetic construct
  source 1..20: mol_type = other RNA
atcctgcaagtagcagactc

SEQ ID NO: 1031 - RNA, 20 nt, synthetic construct
  source 1..20: mol_type = other RNA
taaaatataaactgctcttg

SEQ ID NO: 1032 - RNA, 20 nt, synthetic construct
  source 1..20: mol_type = other RNA
taaaaaaaaaatttagtgcc

SEQ ID NO: 1033 - RNA, 20 nt, synthetic construct
  source 1..20: mol_type = other RNA
aaaatttagtgccaggttta

SEQ ID NO: 1034 - RNA, 20 nt, synthetic construct
  source 1..20: mol_type = other RNA
agcacttcactccataaacc

SEQ ID NO: 1035 - RNA, 20 nt, synthetic construct
  source 1..20: mol_type = other RNA
tgctgaaactacattttctg

SEQ ID NO: 1036 - RNA, 20 nt, synthetic construct
  source 1..20: mol_type = other RNA
gctgaaactacattttctgt

SEQ ID NO: 1037 - RNA, 20 nt, synthetic construct
  source 1..20: mol_type = other RNA
acataaaaaattcttcaaag

SEQ ID NO: 1038 - RNA, 20 nt, synthetic construct
  source 1..20: mol_type = other RNA
aacataaaaaattcttcaaa

SEQ ID NO: 1039 - RNA, 20 nt, synthetic construct
  source 1..20: mol_type = other RNA
gaacataaaaaattcttcaa

SEQ ID NO: 1040 - RNA, 20 nt, synthetic construct
  source 1..20: mol_type = other RNA
gggagatcaaatttttaact

SEQ ID NO: 1041 - RNA, 20 nt, synthetic construct
  source 1..20: mol_type = other RNA
atgaaagctcttactctgta

SEQ ID NO: 1042 - RNA, 20 nt, synthetic construct
  source 1..20: mol_type = other RNA
aatgaaagctcttactctgt

SEQ ID NO: 1043 - RNA, 20 nt, synthetic construct
  source 1..20: mol_type = other RNA
ataaaaccattttatagacc

SEQ ID NO: 1044 - RNA, 20 nt, synthetic construct
  source 1..20: mol_type = other RNA
ttgatacctggtctataaaa

SEQ ID NO: 1045 - RNA, 20 nt, synthetic construct
  source 1..20: mol_type = other RNA
agaccaggtatcaacattta

SEQ ID NO: 1046 - RNA, 20 nt, synthetic construct
  source 1..20: mol_type = other RNA
ccaggtatcaacatttacgg

SEQ ID NO: 1047 - RNA, 20 nt, synthetic construct
  source 1..20: mol_type = other RNA
acacactctttcacatttct

SEQ ID NO: 1048 - RNA, 20 nt, synthetic construct
  source 1..20: mol_type = other RNA
cacacactctttcacatttc

SEQ ID NO: 1049 - RNA, 20 nt, synthetic construct
  source 1..20: mol_type = other RNA
atgtgaaagagtgtgtgaga

SEQ ID NO: 1050 - RNA, 20 nt, synthetic construct
  source 1..20: mol_type = other RNA
tgtgaaagagtgtgtgagat

SEQ ID NO: 1051 - RNA, 20 nt, synthetic construct
  source 1..20: mol_type = other RNA
tgcctctagagacttatctt

SEQ ID NO: 1052 - RNA, 20 nt, synthetic construct
  source 1..20: mol_type = other RNA
ttccaaagataagtctctag

SEQ ID NO: 1053 - RNA, 20 nt, synthetic construct
  source 1..20: mol_type = other RNA
ggaactttcccagtgatctg

SEQ ID NO: 1054 - RNA, 20 nt, synthetic construct
  source 1..20: mol_type = other RNA
attgtggtccacagatcact

SEQ ID NO: 1055 - RNA, 20 nt, synthetic construct
  source 1..20: mol_type = other RNA
cattgtggtccacagatcac

SEQ ID NO: 1056 - RNA, 20 nt, synthetic construct
  source 1..20: mol_type = other RNA
gagggtgtgagcagaaaagc

SEQ ID NO: 1057 - RNA, 20 nt, synthetic construct
  source 1..20: mol_type = other RNA
ggagggtgtgagcagaaaag

SEQ ID NO: 1058 - RNA, 20 nt, synthetic construct
  source 1..20: mol_type = other RNA
aaatatagtgtggaagggga

SEQ ID NO: 1059 - RNA, 20 nt, synthetic construct
  source 1..20: mol_type = other RNA
aaaatatagtgtggaagggg

SEQ ID NO: 1060 - RNA, 20 nt, synthetic construct
  source 1..20: mol_type = other RNA
aaaaaaatatagtgtggaag

SEQ ID NO: 1061 - RNA, 20 nt, synthetic construct
  source 1..20: mol_type = other RNA
taaaaaaatatagtgtggaa

SEQ ID NO: 1062 - RNA, 20 nt, synthetic construct
  source 1..20: mol_type = other RNA
ttaaaaaaatatagtgtgga

SEQ ID NO: 1063 - RNA, 20 nt, synthetic construct
  source 1..20: mol_type = other RNA
ctttttaaaaaaatatagtg

SEQ ID NO: 1064 - RNA, 20 nt, synthetic construct
  source 1..20: mol_type = other RNA
ttgtaactacatgctaattc

SEQ ID NO: 1065 - RNA, 20 nt, synthetic construct
  source 1..20: mol_type = other RNA
aacaatgaaaggtcacaact

SEQ ID NO: 1066 - RNA, 20 nt, synthetic construct
  source 1..20: mol_type = other RNA
gggaaaggagaaacaatgaa

SEQ ID NO: 1067 - RNA, 20 nt, synthetic construct
  source 1..20: mol_type = other RNA
aaacaaatgaaaaatgggaa

SEQ ID NO: 1068 - RNA, 20 nt, synthetic construct
  source 1..20: mol_type = other RNA
tcataaaacaaatgaaaaat

SEQ ID NO: 1069 - RNA, 20 nt, synthetic construct
  source 1..20: mol_type = other RNA
gtcataaaacaaatgaaaaa

SEQ ID NO: 1070 - RNA, 20 nt, synthetic construct
  source 1..20: mol_type = other RNA
tttgttttatgactaagtaa

SEQ ID NO: 1071 - RNA, 20 nt, synthetic construct
  source 1..20: mol_type = other RNA
cttaaataaaataatacagt

SEQ ID NO: 1072 - RNA, 20 nt, synthetic construct
  source 1..20: mol_type = other RNA
aaataaaataatacagtagg

SEQ ID NO: 1073 - RNA, 20 nt, synthetic construct
  source 1..20: mol_type = other RNA
aatacagtaggaggcagcaa

SEQ ID NO: 1074 - RNA, 20 nt, synthetic construct
  source 1..20: mol_type = other RNA
ctttaaaacaatgctaaaaa

SEQ ID NO: 1075 - RNA, 20 nt, synthetic construct
  source 1..20: mol_type = other RNA
tttaaaacaatgctaaaaaa

SEQ ID NO: 1076 - RNA, 20 nt, synthetic construct
  source 1..20: mol_type = other RNA
tctagaaatactattaacat

SEQ ID NO: 1077 - RNA, 20 nt, synthetic construct
  source 1..20: mol_type = other RNA
gagtacagaaacacactaca

SEQ ID NO: 1078 - RNA, 20 nt, synthetic construct
  source 1..20: mol_type = other RNA
gtactccccttgtgcatttt

SEQ ID NO: 1079 - RNA, 20 nt, synthetic construct
  source 1..20: mol_type = other RNA
tttgacctaaaatgcacaag

SEQ ID NO: 1080 - RNA, 20 nt, synthetic construct
  source 1..20: mol_type = other RNA
ctttgacctaaaatgcacaa

SEQ ID NO: 1081 - RNA, 20 nt, synthetic construct
  source 1..20: mol_type = other RNA
actttgacctaaaatgcaca

SEQ ID NO: 1082 - RNA, 20 nt, synthetic construct
  source 1..20: mol_type = other RNA
gcattttaggtcaaagttaa

SEQ ID NO: 1083 - RNA, 20 nt, synthetic construct
  source 1..20: mol_type = other RNA
atcttttgtcacttagcgca

SEQ ID NO: 1084 - RNA, 20 nt, synthetic construct
  source 1..20: mol_type = other RNA
tcttttgtcacttagcgcat

SEQ ID NO: 1085 - RNA, 20 nt, synthetic construct
  source 1..20: mol_type = other RNA
agagtcttttacatgagtgc

SEQ ID NO: 1086 - RNA, 20 nt, synthetic construct
  source 1..20: mol_type = other RNA
aagactctcctgcaatttgc

SEQ ID NO: 1087 - RNA, 20 nt, synthetic construct
  source 1..20: mol_type = other RNA
agactctcctgcaatttgca

SEQ ID NO: 1088 - RNA, 20 nt, synthetic construct
  source 1..20: mol_type = other RNA
ctctcctgcaatttgcaggg

SEQ ID NO: 1089 - RNA, 20 nt, synthetic construct
  source 1..20: mol_type = other RNA
gcaatttgcagggtggcccg

SEQ ID NO: 1090 - RNA, 20 nt, synthetic construct
  source 1..20: mol_type = other RNA
cgggccaccctgcaaattgc

SEQ ID NO: 1091 - RNA, 20 nt, synthetic construct
  source 1..20: mol_type = other RNA
gcagggtggcccgaggaagc

SEQ ID NO: 1092 - RNA, 20 nt, synthetic construct
  source 1..20: mol_type = other RNA
cagggtggcccgaggaagca

SEQ ID NO: 1093 - RNA, 20 nt, synthetic construct
  source 1..20: mol_type = other RNA
caatggctccctgcttcctc

SEQ ID NO: 1094 - RNA, 20 nt, synthetic construct
  source 1..20: mol_type = other RNA
gcaatggctccctgcttcct

SEQ ID NO: 1095 - RNA, 20 nt, synthetic construct
  source 1..20: mol_type = other RNA
aatgggctctgcaagggcaa

SEQ ID NO: 1096 - RNA, 20 nt, synthetic construct
  source 1..20: mol_type = other RNA
gcagagcccattgctgtctt

SEQ ID NO: 1097 - RNA, 20 nt, synthetic construct
  source 1..20: mol_type = other RNA
agacagcaatgggctctgca

SEQ ID NO: 1098 - RNA, 20 nt, synthetic construct
  source 1..20: mol_type = other RNA
aaatgtccaaagacagcaat

SEQ ID NO: 1099 - RNA, 20 nt, synthetic construct
  source 1..20: mol_type = other RNA
taaatgtccaaagacagcaa

SEQ ID NO: 1100 - RNA, 20 nt, synthetic construct
  source 1..20: mol_type = other RNA
tttaattgttgaaatgtatt

SEQ ID NO: 1101 - RNA, 20 nt, synthetic construct
  source 1..20: mol_type = other RNA
aattgttgaaatgtattagg

SEQ ID NO: 1102 - RNA, 20 nt, synthetic construct
  source 1..20: mol_type = other RNA
ctaatcaatagcctgtaatt

SEQ ID NO: 1103 - RNA, 20 nt, synthetic construct
  source 1..20: mol_type = other RNA
taatcaatagcctgtaattt

SEQ ID NO: 1104 - RNA, 20 nt, synthetic construct
  source 1..20: mol_type = other RNA
aattacaggctattgattag

SEQ ID NO: 1105 - RNA, 20 nt, synthetic construct
  source 1..20: mol_type = other RNA
gtttttacagcccaaattac

SEQ ID NO: 1106 - RNA, 20 nt, synthetic construct
  source 1..20: mol_type = other RNA
agaacatagctcaaaataag

SEQ ID NO: 1107 - RNA, 20 nt, synthetic construct
  source 1..20: mol_type = other RNA
ctaactacagaagatgacat

SEQ ID NO: 1108 - RNA, 20 nt, synthetic construct
  source 1..20: mol_type = other RNA
tcttctgtagttagtagaag

SEQ ID NO: 1109 - RNA, 20 nt, synthetic construct
  source 1..20: mol_type = other RNA
tgttttttgtttgttttacc

SEQ ID NO: 1110 - RNA, 20 nt, synthetic construct
  source 1..20: mol_type = other RNA
gttttttgtttgttttacct

SEQ ID NO: 1111 - RNA, 20 nt, synthetic construct
  source 1..20: mol_type = other RNA
ttttttgtttgttttacctg

SEQ ID NO: 1112 - RNA, 20 nt, synthetic construct
  source 1..20: mol_type = other RNA
tttttgtttgttttacctgg

SEQ ID NO: 1113 - RNA, 20 nt, synthetic construct
  source 1..20: mol_type = other RNA
gttttacctgggggcaatgt

SEQ ID NO: 1114 - RNA, 20 nt, synthetic construct
  source 1..20: mol_type = other RNA
gggcaatgtaggtgaccatt

SEQ ID NO: 1115 - RNA, 20 nt, synthetic construct
  source 1..20: mol_type = other RNA
atttggacacctttttcaca

SEQ ID NO: 1116 - RNA, 20 nt, synthetic construct
  source 1..20: mol_type = other RNA
tttggacacctttttcacat

SEQ ID NO: 1117 - RNA, 20 nt, synthetic construct
  source 1..20: mol_type = other RNA
atgtgaaaaaggtgtccaaa

SEQ ID NO: 1118 - RNA, 20 nt, synthetic construct
  source 1..20: mol_type = other RNA
aaaagtgtcccatgtgaaaa

SEQ ID NO: 1119 - RNA, 20 nt, synthetic construct
  source 1..20: mol_type = other RNA
gtgtgtgtttgtttttgaga

SEQ ID NO: 1120 - RNA, 20 nt, synthetic construct
  source 1..20: mol_type = other RNA
cggagtcttgctctgtcacc

SEQ ID NO: 1121 - RNA, 20 nt, synthetic construct
  source 1..20: mol_type = other RNA
gtcaccaggctgaagtgcag

SEQ ID NO: 1122 - RNA, 20 nt, synthetic construct
  source 1..20: mol_type = other RNA
tgcgccactgcacttcagcc

SEQ ID NO: 1123 - RNA, 20 nt, synthetic construct
  source 1..20: mol_type = other RNA
ggcggaggttgcagtgagct

SEQ ID NO: 1124 - RNA, 20 nt, synthetic construct
  source 1..20: mol_type = other RNA
aggcggaggttgcagtgagc

SEQ ID NO: 1125 - RNA, 20 nt, synthetic construct
  source 1..20: mol_type = other RNA
cactgcaacctccgcctccc

SEQ ID NO: 1126 - RNA, 20 nt, synthetic construct
  source 1..20: mol_type = other RNA
cacttgaacctgggaggcgg

SEQ ID NO: 1127 - RNA, 20 nt, synthetic construct
  source 1..20: mol_type = other RNA
aatcacttgaacctgggagg

SEQ ID NO: 1128 - RNA, 20 nt, synthetic construct
  source 1..20: mol_type = other RNA
gagaatcacttgaacctggg

SEQ ID NO: 1129 - RNA, 20 nt, synthetic construct
  source 1..20: mol_type = other RNA
caggagaatcacttgaacct

SEQ ID NO: 1130 - RNA, 20 nt, synthetic construct
  source 1..20: mol_type = other RNA
gcaggagaatcacttgaacc

SEQ ID NO: 1131 - RNA, 20 nt, synthetic construct
  source 1..20: mol_type = other RNA
gcctcagcctcttgagtagc

SEQ ID NO: 1132 - RNA, 20 nt, synthetic construct
  source 1..20: mol_type = other RNA
cctcagcctcttgagtagct

SEQ ID NO: 1133 - RNA, 20 nt, synthetic construct
  source 1..20: mol_type = other RNA
gctactcaagaggctgaggc

SEQ ID NO: 1134 - RNA, 20 nt, synthetic construct
  source 1..20: mol_type = other RNA
cccagctactcaagaggctg

SEQ ID NO: 1135 - RNA, 20 nt, synthetic construct
  source 1..20: mol_type = other RNA
tcttgagtagctgggattac

SEQ ID NO: 1136 - RNA, 20 nt, synthetic construct
  source 1..20: mol_type = other RNA
tgtaatcccagctactcaag

SEQ ID NO: 1137 - RNA, 20 nt, synthetic construct
  source 1..20: mol_type = other RNA
aactagctgggtgtggttgc

SEQ ID NO: 1138 - RNA, 20 nt, synthetic construct
  source 1..20: mol_type = other RNA
aatacaaaactagctgggtg

SEQ ID NO: 1139 - RNA, 20 nt, synthetic construct
  source 1..20: mol_type = other RNA
ctaaaaatacaaaactagct

SEQ ID NO: 1140 - RNA, 20 nt, synthetic construct
  source 1..20: mol_type = other RNA
actaaaaatacaaaactagc

SEQ ID NO: 1141 - RNA, 20 nt, synthetic construct
  source 1..20: mol_type = other RNA
ttttgtatttttagttgaga

SEQ ID NO: 1142 - RNA, 20 nt, synthetic construct
  source 1..20: mol_type = other RNA
tttgtatttttagttgagat

SEQ ID NO: 1143 - RNA, 20 nt, synthetic construct
  source 1..20: mol_type = other RNA
ttgtatttttagttgagatg

SEQ ID NO: 1144 - RNA, 20 nt, synthetic construct
  source 1..20: mol_type = other RNA
ggggtttcaccatattgtcc

SEQ ID NO: 1145 - RNA, 20 nt, synthetic construct
  source 1..20: mol_type = other RNA
cgagatcatcctggacaata

SEQ ID NO: 1146 - RNA, 20 nt, synthetic construct
  source 1..20: mol_type = other RNA
tcaggaaatcgagatcatcc

SEQ ID NO: 1147 - RNA, 20 nt, synthetic construct
  source 1..20: mol_type = other RNA
actctgtgatctgcctgcct

SEQ ID NO: 1148 - RNA, 20 nt, synthetic construct
  source 1..20: mol_type = other RNA
ggcaggcagatcacagagtc

SEQ ID NO: 1149 - RNA, 20 nt, synthetic construct
  source 1..20: mol_type = other RNA
gcctcggcctcccaaagtgc

SEQ ID NO: 1150 - RNA, 20 nt, synthetic construct
  source 1..20: mol_type = other RNA
cctcggcctcccaaagtgct

SEQ ID NO: 1151 - RNA, 20 nt, synthetic construct
  source 1..20: mol_type = other RNA
gcactttgggaggccgaggc

SEQ ID NO: 1152 - RNA, 20 nt, synthetic construct
  source 1..20: mol_type = other RNA
cccagcactttgggaggccg

SEQ ID NO: 1153 - RNA, 20 nt, synthetic construct
  source 1..20: mol_type = other RNA
tcccaaagtgctgggattac

SEQ ID NO: 1154 - RNA, 20 nt, synthetic construct
  source 1..20: mol_type = other RNA
tgtaatcccagcactttggg

SEQ ID NO: 1155 - RNA, 20 nt, synthetic construct
  source 1..20: mol_type = other RNA
acctgtaatcccagcacttt

SEQ ID NO: 1156 - RNA, 20 nt, synthetic construct
  source 1..20: mol_type = other RNA
cacctgtaatcccagcactt

SEQ ID NO: 1157 - RNA, 20 nt, synthetic construct
  source 1..20: mol_type = other RNA
caggtgtgagcctctgcgcc

SEQ ID NO: 1158 - RNA, 20 nt, synthetic construct
  source 1..20: mol_type = other RNA
agcctctgcgcctggccgca

SEQ ID NO: 1159 - RNA, 20 nt, synthetic construct
  source 1..20: mol_type = other RNA
gcctctgcgcctggccgcat

SEQ ID NO: 1160 - RNA, 20 nt, synthetic construct
  source 1..20: mol_type = other RNA
tcccatgcggccaggcgcag

SEQ ID NO: 1161 - RNA, 20 nt, synthetic construct
  source 1..20: mol_type = other RNA
aaaatgtctcccatgcggcc

SEQ ID NO: 1162 - RNA, 20 nt, synthetic construct
  source 1..20: mol_type = other RNA
atttaaaaatgtctcccatg

SEQ ID NO: 1163 - RNA, 20 nt, synthetic construct
  source 1..20: mol_type = other RNA
aatgtgtagactttgactcc

SEQ ID NO: 1164 - RNA, 20 nt, synthetic construct
  source 1..20: mol_type = other RNA
actccaggagttagtaccat

SEQ ID NO: 1165 - RNA, 20 nt, synthetic construct
  source 1..20: mol_type = other RNA
ctccaggagttagtaccatt

SEQ ID NO: 1166 - RNA, 20 nt, synthetic construct
  source 1..20: mol_type = other RNA
ttcccaatggtactaactcc

SEQ ID NO: 1167 - RNA, 20 nt, synthetic construct
  source 1..20: mol_type = other RNA
gcagtcacaggtgttcccaa

SEQ ID NO: 1168 - RNA, 20 nt, synthetic construct
  source 1..20: mol_type = other RNA
cctgtgactgcttccgctaa

SEQ ID NO: 1169 - RNA, 20 nt, synthetic construct
  source 1..20: mol_type = other RNA
ctgtgactgcttccgctaaa

SEQ ID NO: 1170 - RNA, 20 nt, synthetic construct
  source 1..20: mol_type = other RNA
cctttagcggaagcagtcac

SEQ ID NO: 1171 - RNA, 20 nt, synthetic construct
  source 1..20: mol_type = other RNA
tttgctagtgtaccctttag

SEQ ID NO: 1172 - RNA, 20 nt, synthetic construct
  source 1..20: mol_type = other RNA
gttttaaacacctcatataa

SEQ ID NO: 1173 - RNA, 20 nt, synthetic construct
  source 1..20: mol_type = other RNA
tgaattaatacctttatatg

SEQ ID NO: 1174 - RNA, 20 nt, synthetic construct
  source 1..20: mol_type = other RNA
attcagttgatttatccaaa

SEQ ID NO: 1175 - RNA, 20 nt, synthetic construct
  source 1..20: mol_type = other RNA
aagaattagtgtcttccttt

SEQ ID NO: 1176 - RNA, 20 nt, synthetic construct
  source 1..20: mol_type = other RNA
agacactaattcttattttg

SEQ ID NO: 1177 - RNA, 20 nt, synthetic construct
  source 1..20: mol_type = other RNA
aaaaagagctaaaagagaag

SEQ ID NO: 1178 - RNA, 20 nt, synthetic construct
  source 1..20: mol_type = other RNA
aaaaaagagctaaaagagaa

SEQ ID NO: 1179 - RNA, 20 nt, synthetic construct
  source 1..20: mol_type = other RNA
aaaaaaagagctaaaagaga

SEQ ID NO: 1180 - RNA, 20 nt, synthetic construct
  source 1..20: mol_type = other RNA
attaaaaaaaaacttttaag

SEQ ID NO: 1181 - RNA, 20 nt, synthetic construct
  source 1..20: mol_type = other RNA
ttttttttaatctgttttct

SEQ ID NO: 1182 - RNA, 20 nt, synthetic construct
  source 1..20: mol_type = other RNA
tttttttaatctgttttcta

SEQ ID NO: 1183 - RNA, 20 nt, synthetic construct
  source 1..20: mol_type = other RNA
ttttttaatctgttttctag

SEQ ID NO: 1184 - RNA, 20 nt, synthetic construct
  source 1..20: mol_type = other RNA
tttaatctgttttctagggg

SEQ ID NO: 1185 - RNA, 20 nt, synthetic construct
  source 1..20: mol_type = other RNA
tttctaggggaggtcatgct

SEQ ID NO: 1186 - RNA, 20 nt, synthetic construct
  source 1..20: mol_type = other RNA
gttaattgttgctaagtaaa

SEQ ID NO: 1187 - RNA, 20 nt, synthetic construct
  source 1..20: mol_type = other RNA
ggcagaaaaataataatcaa

SEQ ID NO: 1188 - RNA, 20 nt, synthetic construct
  source 1..20: mol_type = other RNA
gcctttatacaatgtgtttt

SEQ ID NO: 1189 - RNA, 20 nt, synthetic construct
  source 1..20: mol_type = other RNA
gcctaaaacacattgtataa

SEQ ID NO: 1190 - RNA, 20 nt, synthetic construct
  source 1..20: mol_type = other RNA
tagacattttcccattacaa

SEQ ID NO: 1191 - RNA, 20 nt, synthetic construct
  source 1..20: mol_type = other RNA
ctgatagtgtcctttgtaat

SEQ ID NO: 1192 - RNA, 20 nt, synthetic construct
  source 1..20: mol_type = other RNA
actgatagtgtcctttgtaa

SEQ ID NO: 1193 - RNA, 20 nt, synthetic construct
  source 1..20: mol_type = other RNA
acactatcagttcttcagta

SEQ ID NO: 1194 - RNA, 20 nt, synthetic construct
  source 1..20: mol_type = other RNA
agagtcaagaaaacacacat

SEQ ID NO: 1195 - RNA, 20 nt, synthetic construct
  source 1..20: mol_type = other RNA
cggatcttcctacctttctg

SEQ ID NO: 1196 - RNA, 20 nt, synthetic construct
  source 1..20: mol_type = other RNA
ggatcttcctacctttctgt

SEQ ID NO: 1197 - RNA, 20 nt, synthetic construct
  source 1..20: mol_type = other RNA
gatcttcctacctttctgtg

SEQ ID NO: 1198 - RNA, 20 nt, synthetic construct
  source 1..20: mol_type = other RNA
atcttcctacctttctgtgg

SEQ ID NO: 1199 - RNA, 20 nt, synthetic construct
  source 1..20: mol_type = other RNA
cctttctgtgggggtgtttg

SEQ ID NO: 1200 - RNA, 20 nt, synthetic construct
  source 1..20: mol_type = other RNA
aaacacccccacagaaaggt

SEQ ID NO: 1201 - RNA, 20 nt, synthetic construct
  source 1..20: mol_type = other RNA
cctcaaacacccccacagaa

SEQ ID NO: 1202 - RNA, 20 nt, synthetic construct
  source 1..20: mol_type = other RNA
gtaatgattctgttgtaaaa

SEQ ID NO: 1203 - RNA, 20 nt, synthetic construct
  source 1..20: mol_type = other RNA
taatgattctgttgtaaaat

SEQ ID NO: 1204 - RNA, 20 nt, synthetic construct
  source 1..20: mol_type = other RNA
aatgggaagtgtgacattga

SEQ ID NO: 1205 - RNA, 20 nt, synthetic construct
  source 1..20: mol_type = other RNA
cttaaaatactgtcttaagc

SEQ ID NO: 1206 - RNA, 20 nt, synthetic construct
  source 1..20: mol_type = other RNA
tcttaagctggcaaaactcc

SEQ ID NO: 1207 - RNA, 20 nt, synthetic construct
  source 1..20: mol_type = other RNA
tatgtcaggtggaggatgcc

SEQ ID NO: 1208 - RNA, 20 nt, synthetic construct
  source 1..20: mol_type = other RNA
aactggtttatgtcaggtgg

SEQ ID NO: 1209 - RNA, 20 nt, synthetic construct
  source 1..20: mol_type = other RNA
gtgaactggtttatgtcagg

SEQ ID NO: 1210 - RNA, 20 nt, synthetic construct
  source 1..20: mol_type = other RNA
tctgtgaactggtttatgtc

SEQ ID NO: 1211 - RNA, 20 nt, synthetic construct
  source 1..20: mol_type = other RNA
ggctggaatgttctgtgaac

SEQ ID NO: 1212 - RNA, 20 nt, synthetic construct
  source 1..20: mol_type = other RNA
attccagcctagatctgaaa

SEQ ID NO: 1213 - RNA, 20 nt, synthetic construct
  source 1..20: mol_type = other RNA
ttaccatttcagatctaggc

SEQ ID NO: 1214 - RNA, 20 nt, synthetic construct
  source 1..20: mol_type = other RNA
atctgaaatggtaatttttt

SEQ ID NO: 1215 - RNA, 20 nt, synthetic construct
  source 1..20: mol_type = other RNA
tggtaatttttttggaactt

SEQ ID NO: 1216 - RNA, 20 nt, synthetic construct
  source 1..20: mol_type = other RNA
aatttttttggaactttggt

SEQ ID NO: 1217 - RNA, 20 nt, synthetic construct
  source 1..20: mol_type = other RNA
tccctccagttcctctgcct

SEQ ID NO: 1218 - RNA, 20 nt, synthetic construct
  source 1..20: mol_type = other RNA
ggcagaggaactggagggaa

SEQ ID NO: 1219 - RNA, 20 nt, synthetic construct
  source 1..20: mol_type = other RNA
accaaggcagaggaactgga

SEQ ID NO: 1220 - RNA, 20 nt, synthetic construct
  source 1..20: mol_type = other RNA
aaccaaggcagaggaactgg

SEQ ID NO: 1221 - RNA, 20 nt, synthetic construct
  source 1..20: mol_type = other RNA
gtaaaccaaggcagaggaac

SEQ ID NO: 1222 - RNA, 20 nt, synthetic construct
  source 1..20: mol_type = other RNA
ctctgccttggtttacctaa

SEQ ID NO: 1223 - RNA, 20 nt, synthetic construct
  source 1..20: mol_type = other RNA
tctgccttggtttacctaaa

SEQ ID NO: 1224 - RNA, 20 nt, synthetic construct
  source 1..20: mol_type = other RNA
ctttaggtaaaccaaggcag

SEQ ID NO: 1225 - RNA, 20 nt, synthetic construct
  source 1..20: mol_type = other RNA
tggtttacctaaagggattt

SEQ ID NO: 1226 - RNA, 20 nt, synthetic construct
  source 1..20: mol_type = other RNA
aaatccctttaggtaaacca

SEQ ID NO: 1227 - RNA, 20 nt, synthetic construct
  source 1..20: mol_type = other RNA
aggaacaccaaaatcccttt

SEQ ID NO: 1228 - RNA, 20 nt, synthetic construct
  source 1..20: mol_type = other RNA
ttggtgttcctgtgtgtgac

SEQ ID NO: 1229 - RNA, 20 nt, synthetic construct
  source 1..20: mol_type = other RNA
ttcctgtgtgtgactggaag

SEQ ID NO: 1230 - RNA, 20 nt, synthetic construct
  source 1..20: mol_type = other RNA
agccacttccagtcacacac

SEQ ID NO: 1231 - RNA, 20 nt, synthetic construct
  source 1..20: mol_type = other RNA
agtggctgtctctattgact

SEQ ID NO: 1232 - RNA, 20 nt, synthetic construct
  source 1..20: mol_type = other RNA
ctctattgactaggaagaac

SEQ ID NO: 1233 - RNA, 20 nt, synthetic construct
  source 1..20: mol_type = other RNA
taggaagaactggtgagaag

SEQ ID NO: 1234 - RNA, 20 nt, synthetic construct
  source 1..20: mol_type = other RNA
aggaagaactggtgagaagt

SEQ ID NO: 1235 - RNA, 20 nt, synthetic construct
  source 1..20: mol_type = other RNA
agtgggaccacagtgtattc

SEQ ID NO: 1236 - RNA, 20 nt, synthetic construct
  source 1..20: mol_type = other RNA
cagtgtattcaggatcaaag

SEQ ID NO: 1237 - RNA, 20 nt, synthetic construct
  source 1..20: mol_type = other RNA
agtgtattcaggatcaaagt

SEQ ID NO: 1238 - RNA, 20 nt, synthetic construct
  source 1..20: mol_type = other RNA
ctttgatcctgaatacactg

SEQ ID NO: 1239 - RNA, 20 nt, synthetic construct
  source 1..20: mol_type = other RNA
tattcaggatcaaagtgggg

SEQ ID NO: 1240 - RNA, 20 nt, synthetic construct
  source 1..20: mol_type = other RNA
aggacatgagtccctttaag

SEQ ID NO: 1241 - RNA, 20 nt, synthetic construct
  source 1..20: mol_type = other RNA
ggacatgagtccctttaaga

SEQ ID NO: 1242 - RNA, 20 nt, synthetic construct
  source 1..20: mol_type = other RNA
atgagtccctttaagagggt

SEQ ID NO: 1243 - RNA, 20 nt, synthetic construct
  source 1..20: mol_type = other RNA
tattcacctaccctcttaaa

SEQ ID NO: 1244 - RNA, 20 nt, synthetic construct
  source 1..20: mol_type = other RNA
gtattcacctaccctcttaa

SEQ ID NO: 1245 - RNA, 20 nt, synthetic construct
  source 1..20: mol_type = other RNA
atacactcaagtcccgattc

SEQ ID NO: 1246 - RNA, 20 nt, synthetic construct
  source 1..20: mol_type = other RNA
ctggacacaataccagaatc

SEQ ID NO: 1247 - RNA, 20 nt, synthetic construct
  source 1..20: mol_type = other RNA
tctggacacaataccagaat

SEQ ID NO: 1248 - RNA, 20 nt, synthetic construct
  source 1..20: mol_type = other RNA
tattgtgtccagaatccaac

SEQ ID NO: 1249 - RNA, 20 nt, synthetic construct
  source 1..20: mol_type = other RNA
tgatctgtcctgttggattc

SEQ ID NO: 1250 - RNA, 20 nt, synthetic construct
  source 1..20: mol_type = other RNA
acaggacagatcatttctga

SEQ ID NO: 1251 - RNA, 20 nt, synthetic construct
  source 1..20: mol_type = other RNA
caggacagatcatttctgat

SEQ ID NO: 1252 - RNA, 20 nt, synthetic construct
  source 1..20: mol_type = other RNA
tcagaaatgatctgtcctgt

SEQ ID NO: 1253 - RNA, 20 nt, synthetic construct
  source 1..20: mol_type = other RNA
cagatcatttctgatgggta

SEQ ID NO: 1254 - RNA, 20 nt, synthetic construct
  source 1..20: mol_type = other RNA
atggagacatctctgaacct

SEQ ID NO: 1255 - RNA, 20 nt, synthetic construct
  source 1..20: mol_type = other RNA
ggatggtcagttcattgcct

SEQ ID NO: 1256 - RNA, 20 nt, synthetic construct
  source 1..20: mol_type = other RNA
caatgaactgaccatcccct

SEQ ID NO: 1257 - RNA, 20 nt, synthetic construct
  source 1..20: mol_type = other RNA
aaggagacaggcccagggga

SEQ ID NO: 1258 - RNA, 20 nt, synthetic construct
  source 1..20: mol_type = other RNA
gggcctgtctccttcccgtc

SEQ ID NO: 1259 - RNA, 20 nt, synthetic construct
  source 1..20: mol_type = other RNA
acgggaaggagacaggccca

SEQ ID NO: 1260 - RNA, 20 nt, synthetic construct
  source 1..20: mol_type = other RNA
gacgggaaggagacaggccc

SEQ ID NO: 1261 - RNA, 20 nt, synthetic construct
  source 1..20: mol_type = other RNA
ctgtctccttcccgtctgga

SEQ ID NO: 1262 - RNA, 20 nt, synthetic construct
  source 1..20: mol_type = other RNA
tgtctccttcccgtctggaa

SEQ ID NO: 1263 - RNA, 20 nt, synthetic construct
  source 1..20: mol_type = other RNA
gtctccttcccgtctggaag

SEQ ID NO: 1264 - RNA, 20 nt, synthetic construct
  source 1..20: mol_type = other RNA
cttccagacgggaaggagac

SEQ ID NO: 1265 - RNA, 20 nt, synthetic construct
  source 1..20: mol_type = other RNA
aaagccccttccagacggga

SEQ ID NO: 1266 - RNA, 20 nt, synthetic construct
  source 1..20: mol_type = other RNA
ctacaaagccccttccagac

SEQ ID NO: 1267 - RNA, 20 nt, synthetic construct
  source 1..20: mol_type = other RNA
tctacaaagccccttccaga

SEQ ID NO: 1268 - RNA, 20 nt, synthetic construct
  source 1..20: mol_type = other RNA
aggggctttgtagacaccct

SEQ ID NO: 1269 - RNA, 20 nt, synthetic construct
  source 1..20: mol_type = other RNA
ggggctttgtagacaccctc

SEQ ID NO: 1270 - RNA, 20 nt, synthetic construct
  source 1..20: mol_type = other RNA
gggctttgtagacaccctcg

SEQ ID NO: 1271 - RNA, 20 nt, synthetic construct
  source 1..20: mol_type = other RNA
taaggcagatcttgccccga

SEQ ID NO: 1272 - RNA, 20 nt, synthetic construct
  source 1..20: mol_type = other RNA
gggcaagatctgccttagat

SEQ ID NO: 1273 - RNA, 20 nt, synthetic construct
  source 1..20: mol_type = other RNA
ggcaagatctgccttagatg

SEQ ID NO: 1274 - RNA, 20 nt, synthetic construct
  source 1..20: mol_type = other RNA
ctctcaggcagccccatcta

SEQ ID NO: 1275 - RNA, 20 nt, synthetic construct
  source 1..20: mol_type = other RNA
tggggctgcctgagagaaag

SEQ ID NO: 1276 - RNA, 20 nt, synthetic construct
  source 1..20: mol_type = other RNA
ggctgcctgagagaaagagg

SEQ ID NO: 1277 - RNA, 20 nt, synthetic construct
  source 1..20: mol_type = other RNA
tgagagaaagaggtggcagt

SEQ ID NO: 1278 - RNA, 20 nt, synthetic construct
  source 1..20: mol_type = other RNA
tactgccacctctttctctc

SEQ ID NO: 1279 - RNA, 20 nt, synthetic construct
  source 1..20: mol_type = other RNA
aggtggcagtaggccttgcc

SEQ ID NO: 1280 - RNA, 20 nt, synthetic construct
  source 1..20: mol_type = other RNA
gacactgtgggcaccaggca

SEQ ID NO: 1281 - RNA, 20 nt, synthetic construct
  source 1..20: mol_type = other RNA
agggagacactgtgggcacc

SEQ ID NO: 1282 - RNA, 20 nt, synthetic construct
  source 1..20: mol_type = other RNA
tggcagcagggagacactgt

SEQ ID NO: 1283 - RNA, 20 nt, synthetic construct
  source 1..20: mol_type = other RNA
ttggcagcagggagacactg

SEQ ID NO: 1284 - RNA, 20 nt, synthetic construct
  source 1..20: mol_type = other RNA
ctccctgctgccaagagctc

SEQ ID NO: 1285 - RNA, 20 nt, synthetic construct
  source 1..20: mol_type = other RNA
tccctgctgccaagagctct

SEQ ID NO: 1286 - RNA, 20 nt, synthetic construct
  source 1..20: mol_type = other RNA
acccagagctcttggcagca

SEQ ID NO: 1287 - RNA, 20 nt, synthetic construct
  source 1..20: mol_type = other RNA
tacccagagctcttggcagc

SEQ ID NO: 1288 - RNA, 20 nt, synthetic construct
  source 1..20: mol_type = other RNA
atctcagtacccagagctct

SEQ ID NO: 1289 - RNA, 20 nt, synthetic construct
  source 1..20: mol_type = other RNA
gataagcttgcacattctca

SEQ ID NO: 1290 - RNA, 20 nt, synthetic construct
  source 1..20: mol_type = other RNA
agagattttgaccgcagagc

SEQ ID NO: 1291 - RNA, 20 nt, synthetic construct
  source 1..20: mol_type = other RNA
cgcagagctggttgtgttaa

SEQ ID NO: 1292 - RNA, 20 nt, synthetic construct
  source 1..20: mol_type = other RNA
ctttaacacaaccagctctg

SEQ ID NO: 1293 - RNA, 20 nt, synthetic construct
  source 1..20: mol_type = other RNA
tatgaatgcatgactccaca

SEQ ID NO: 1294 - RNA, 20 nt, synthetic construct
  source 1..20: mol_type = other RNA
gactccacaaggctttcctg

SEQ ID NO: 1295 - RNA, 20 nt, synthetic construct
  source 1..20: mol_type = other RNA
actccacaaggctttcctgt

SEQ ID NO: 1296 - RNA, 20 nt, synthetic construct
  source 1..20: mol_type = other RNA
aggcccacaggaaagccttg

SEQ ID NO: 1297 - RNA, 20 nt, synthetic construct
  source 1..20: mol_type = other RNA
ttcctgtgggcctgcccaga

SEQ ID NO: 1298 - RNA, 20 nt, synthetic construct
  source 1..20: mol_type = other RNA
tgggcctgcccagatggacc

SEQ ID NO: 1299 - RNA, 20 nt, synthetic construct
  source 1..20: mol_type = other RNA
gtccatctgggcaggcccac

SEQ ID NO: 1300 - RNA, 20 nt, synthetic construct
  source 1..20: mol_type = other RNA
gcctgcccagatggacctgg

SEQ ID NO: 1301 - RNA, 20 nt, synthetic construct
  source 1..20: mol_type = other RNA
tccaccaggtccatctgggc

SEQ ID NO: 1302 - RNA, 20 nt, synthetic construct
  source 1..20: mol_type = other RNA
tgcatccaccaggtccatct

SEQ ID NO: 1303 - RNA, 20 nt, synthetic construct
  source 1..20: mol_type = other RNA
gtgcatccaccaggtccatc

SEQ ID NO: 1304 - RNA, 20 nt, synthetic construct
  source 1..20: mol_type = other RNA
acctggtggatgcacctcca

SEQ ID NO: 1305 - RNA, 20 nt, synthetic construct
  source 1..20: mol_type = other RNA
gccatggaggtgcatccacc

SEQ ID NO: 1306 - RNA, 20 nt, synthetic construct
  source 1..20: mol_type = other RNA
acctccatggctgccatgag

SEQ ID NO: 1307 - RNA, 20 nt, synthetic construct
  source 1..20: mol_type = other RNA
accactcatggcagccatgg

SEQ ID NO: 1308 - RNA, 20 nt, synthetic construct
  source 1..20: mol_type = other RNA
ctgaccactcatggcagcca

SEQ ID NO: 1309 - RNA, 20 nt, synthetic construct
  source 1..20: mol_type = other RNA
gtcttgtcactgaccactca

SEQ ID NO: 1310 - RNA, 20 nt, synthetic construct
  source 1..20: mol_type = other RNA
cagtgacaagacataggcta

SEQ ID NO: 1311 - RNA, 20 nt, synthetic construct
  source 1..20: mol_type = other RNA
gacaagacataggctaaggc

SEQ ID NO: 1312 - RNA, 20 nt, synthetic construct
  source 1..20: mol_type = other RNA
gacataggctaaggctggca

SEQ ID NO: 1313 - RNA, 20 nt, synthetic construct
  source 1..20: mol_type = other RNA
acataggctaaggctggcat

SEQ ID NO: 1314 - RNA, 20 nt, synthetic construct
  source 1..20: mol_type = other RNA
cataggctaaggctggcatg

SEQ ID NO: 1315 - RNA, 20 nt, synthetic construct
  source 1..20: mol_type = other RNA
gctaaggctggcatggggac

SEQ ID NO: 1316 - RNA, 20 nt, synthetic construct
  source 1..20: mol_type = other RNA
ctggagtgcatcccagtccc

SEQ ID NO: 1317 - RNA, 20 nt, synthetic construct
  source 1..20: mol_type = other RNA
caagaggatggccggggact

SEQ ID NO: 1318 - RNA, 20 nt, synthetic construct
  source 1..20: mol_type = other RNA
ccccggccatcctcttgtga

SEQ ID NO: 1319 - RNA, 20 nt, synthetic construct
  source 1..20: mol_type = other RNA
ccttcacaagaggatggccg

SEQ ID NO: 1320 - RNA, 20 nt, synthetic construct
  source 1..20: mol_type = other RNA
gccttcacaagaggatggcc

SEQ ID NO: 1321 - RNA, 20 nt, synthetic construct
  source 1..20: mol_type = other RNA
agccttcacaagaggatggc

SEQ ID NO: 1322 - RNA, 20 nt, synthetic construct
  source 1..20: mol_type = other RNA
tcctcttgtgaaggctgtca

SEQ ID NO: 1323 - RNA, 20 nt, synthetic construct
  source 1..20: mol_type = other RNA
tgacagccttcacaagagga

SEQ ID NO: 1324 - RNA, 20 nt, synthetic construct
  source 1..20: mol_type = other RNA
tcttgtgaaggctgtcaagg

SEQ ID NO: 1325 - RNA, 20 nt, synthetic construct
  source 1..20: mol_type = other RNA
cttgtgaaggctgtcaaggt

SEQ ID NO: 1326 - RNA, 20 nt, synthetic construct
  source 1..20: mol_type = other RNA
ttgtgaaggctgtcaaggtg

SEQ ID NO: 1327 - RNA, 20 nt, synthetic construct
  source 1..20: mol_type = other RNA
accttgacagccttcacaag

SEQ ID NO: 1328 - RNA, 20 nt, synthetic construct
  source 1..20: mol_type = other RNA
gtcatatgcagatgaaacct

SEQ ID NO: 1329 - RNA, 20 nt, synthetic construct
  source 1..20: mol_type = other RNA
gcagatgaaacctaggctgc

SEQ ID NO: 1330 - RNA, 20 nt, synthetic construct
  source 1..20: mol_type = other RNA
cagatgaaacctaggctgct

SEQ ID NO: 1331 - RNA, 20 nt, synthetic construct
  source 1..20: mol_type = other RNA
caaagacaacccagcagcct

SEQ ID NO: 1332 - RNA, 20 nt, synthetic construct
  source 1..20: mol_type = other RNA
gttaccttgcctctctgttg

SEQ ID NO: 1333 - RNA, 20 nt, synthetic construct
  source 1..20: mol_type = other RNA
acatcctcaacagagaggca

SEQ ID NO: 1334 - RNA, 20 nt, synthetic construct
  source 1..20: mol_type = other RNA
ctatcacatcctcaacagag

SEQ ID NO: 1335 - RNA, 20 nt, synthetic construct
  source 1..20: mol_type = other RNA
atgtgatagcagcacctaac

SEQ ID NO: 1336 - RNA, 20 nt, synthetic construct
  source 1..20: mol_type = other RNA
aggcaggctatgaacctgtt

SEQ ID NO: 1337 - RNA, 20 nt, synthetic construct
  source 1..20: mol_type = other RNA
gggagaagaggaggggaggc

SEQ ID NO: 1338 - RNA, 20 nt, synthetic construct
  source 1..20: mol_type = other RNA
cattgggagaagaggagggg

SEQ ID NO: 1339 - RNA, 20 nt, synthetic construct
  source 1..20: mol_type = other RNA
tgacattgggagaagaggag

SEQ ID NO: 1340 - RNA, 20 nt, synthetic construct
  source 1..20: mol_type = other RNA
atgacattgggagaagagga

SEQ ID NO: 1341 - RNA, 20 nt, synthetic construct
  source 1..20: mol_type = other RNA
aatgacattgggagaagagg

SEQ ID NO: 1342 - RNA, 20 nt, synthetic construct
  source 1..20: mol_type = other RNA
tgaaatgacattgggagaag

SEQ ID NO: 1343 - RNA, 20 nt, synthetic construct
  source 1..20: mol_type = other RNA
ttaaactgtgaaatgacatt

SEQ ID NO: 1344 - RNA, 20 nt, synthetic construct
  source 1..20: mol_type = other RNA
attaaactgtgaaatgacat

SEQ ID NO: 1345 - RNA, 20 nt, synthetic construct
  source 1..20: mol_type = other RNA
gtttaagcgtatgtttaaga

SEQ ID NO: 1346 - RNA, 20 nt, synthetic construct
  source 1..20: mol_type = other RNA
aacaataggttgcatcttat

SEQ ID NO: 1347 - RNA, 20 nt, synthetic construct
  source 1..20: mol_type = other RNA
acctattgttcccatgcttt

SEQ ID NO: 1348 - RNA, 20 nt, synthetic construct
  source 1..20: mol_type = other RNA
accaaaagcatgggaacaat

SEQ ID NO: 1349 - RNA, 20 nt, synthetic construct
  source 1..20: mol_type = other RNA
atttaatttaccaaaagcat

SEQ ID NO: 1350 - RNA, 20 nt, synthetic construct
  source 1..20: mol_type = other RNA
aatttaatttaccaaaagca

SEQ ID NO: 1351 - RNA, 20 nt, synthetic construct
  source 1..20: mol_type = other RNA
gtctgattgcagtatttaca

SEQ ID NO: 1352 - RNA, 20 nt, synthetic construct
  source 1..20: mol_type = other RNA
aaagacactcaacatttaaa

SEQ ID NO: 1353 - RNA, 20 nt, synthetic construct
  source 1..20: mol_type = other RNA
aaagactaacactttagaca

SEQ ID NO: 1354 - RNA, 20 nt, synthetic construct
  source 1..20: mol_type = other RNA
cgagccttgcaaagcctgac

SEQ ID NO: 1355 - RNA, 20 nt, synthetic construct
  source 1..20: mol_type = other RNA
gtcaggctttgcaaggctcg

SEQ ID NO: 1356 - RNA, 20 nt, synthetic construct
  source 1..20: mol_type = other RNA
atatcctgtcaggctttgca

SEQ ID NO: 1357 - RNA, 20 nt, synthetic construct
  source 1..20: mol_type = other RNA
tcatgtattcagtccactta

SEQ ID NO: 1358 - RNA, 20 nt, synthetic construct
  source 1..20: mol_type = other RNA
catgtattcagtccacttaa

SEQ ID NO: 1359 - RNA, 20 nt, synthetic construct
  source 1..20: mol_type = other RNA
ttcagtccacttaagggcag

SEQ ID NO: 1360 - RNA, 20 nt, synthetic construct
  source 1..20: mol_type = other RNA
tcagtccacttaagggcagt

SEQ ID NO: 1361 - RNA, 20 nt, synthetic construct
  source 1..20: mol_type = other RNA
cagtccacttaagggcagtg

SEQ ID NO: 1362 - RNA, 20 nt, synthetic construct
  source 1..20: mol_type = other RNA
gcttccccactgcccttaag

SEQ ID NO: 1363 - RNA, 20 nt, synthetic construct
  source 1..20: mol_type = other RNA
cagtggggaagcgtttgaga

SEQ ID NO: 1364 - RNA, 20 nt, synthetic construct
  source 1..20: mol_type = other RNA
aagcgtttgagacggagctg

SEQ ID NO: 1365 - RNA, 20 nt, synthetic construct
  source 1..20: mol_type = other RNA
cgtttgagacggagctgtgg

SEQ ID NO: 1366 - RNA, 20 nt, synthetic construct
  source 1..20: mol_type = other RNA
tgtggaggctgaatccttga

SEQ ID NO: 1367 - RNA, 20 nt, synthetic construct
  source 1..20: mol_type = other RNA
ggaggctgaatccttgaagg

SEQ ID NO: 1368 - RNA, 20 nt, synthetic construct
  source 1..20: mol_type = other RNA
ggctgaatccttgaaggagg

SEQ ID NO: 1369 - RNA, 20 nt, synthetic construct
  source 1..20: mol_type = other RNA
cttgaaggaggaggtgagag

SEQ ID NO: 1370 - RNA, 20 nt, synthetic construct
  source 1..20: mol_type = other RNA
ctctctcacctcctccttca

SEQ ID NO: 1371 - RNA, 20 nt, synthetic construct
  source 1..20: mol_type = other RNA
ggaggaggtgagagaggcac

SEQ ID NO: 1372 - RNA, 20 nt, synthetic construct
  source 1..20: mol_type = other RNA
gagaagaggggacatgcact

SEQ ID NO: 1373 - RNA, 20 nt, synthetic construct
  source 1..20: mol_type = other RNA
agagaagaggggacatgcac

SEQ ID NO: 1374 - RNA, 20 nt, synthetic construct
  source 1..20: mol_type = other RNA
actgcatcgggagagaagag

SEQ ID NO: 1375 - RNA, 20 nt, synthetic construct
  source 1..20: mol_type = other RNA
cactgcatcgggagagaaga

SEQ ID NO: 1376 - RNA, 20 nt, synthetic construct
  source 1..20: mol_type = other RNA
acactgcatcgggagagaag

SEQ ID NO: 1377 - RNA, 20 nt, synthetic construct
  source 1..20: mol_type = other RNA
cccgatgcagtgtcattccc

SEQ ID NO: 1378 - RNA, 20 nt, synthetic construct
  source 1..20: mol_type = other RNA
cctgggaatgacactgcatc

SEQ ID NO: 1379 - RNA, 20 nt, synthetic construct
  source 1..20: mol_type = other RNA
acctgggaatgacactgcat

SEQ ID NO: 1380 - RNA, 20 nt, synthetic construct
  source 1..20: mol_type = other RNA
tcattcccaggtgaacctgc

SEQ ID NO: 1381 - RNA, 20 nt, synthetic construct
  source 1..20: mol_type = other RNA
cattcccaggtgaacctgcc

SEQ ID NO: 1382 - RNA, 20 nt, synthetic construct
  source 1..20: mol_type = other RNA
ggtgaacctgccgggctgaa

SEQ ID NO: 1383 - RNA, 20 nt, synthetic construct
  source 1..20: mol_type = other RNA
tcagcccggcaggttcacct

SEQ ID NO: 1384 - RNA, 20 nt, synthetic construct
  source 1..20: mol_type = other RNA
ttcagcccggcaggttcacc

SEQ ID NO: 1385 - RNA, 20 nt, synthetic construct
  source 1..20: mol_type = other RNA
acctgccgggctgaacggcc

SEQ ID NO: 1386 - RNA, 20 nt, synthetic construct
  source 1..20: mol_type = other RNA
gccaggccgttcagcccggc

SEQ ID NO: 1387 - RNA, 20 nt, synthetic construct
  source 1..20: mol_type = other RNA
aggggccaggccgttcagcc

SEQ ID NO: 1388 - RNA, 20 nt, synthetic construct
  source 1..20: mol_type = other RNA
gcctggcccctctattcagt

SEQ ID NO: 1389 - RNA, 20 nt, synthetic construct
  source 1..20: mol_type = other RNA
tccgactgaatagaggggcc

SEQ ID NO: 1390 - RNA, 20 nt, synthetic construct
  source 1..20: mol_type = other RNA
aaaactccgactgaatagag

SEQ ID NO: 1391 - RNA, 20 nt, synthetic construct
  source 1..20: mol_type = other RNA
taaaactccgactgaataga

SEQ ID NO: 1392 - RNA, 20 nt, synthetic construct
  source 1..20: mol_type = other RNA
gtaaaactccgactgaatag

SEQ ID NO: 1393 - RNA, 20 nt, synthetic construct
  source 1..20: mol_type = other RNA
tcggagttttactactccag

SEQ ID NO: 1394 - RNA, 20 nt, synthetic construct
  source 1..20: mol_type = other RNA
tattaaaataaatacaatca

SEQ ID NO: 1395 - RNA, 20 nt, synthetic construct
  source 1..20: mol_type = other RNA
ctattaaaataaatacaatc

SEQ ID NO: 1396 - RNA, 20 nt, synthetic construct
  source 1..20: mol_type = other RNA
tttaaaaaacgcttgtaatc

SEQ ID NO: 1397 - RNA, 20 nt, synthetic construct
  source 1..20: mol_type = other RNA
cttttttatattacccagtt

SEQ ID NO: 1398 - RNA, 20 nt, synthetic construct
  source 1..20: mol_type = other RNA
ttttttatattacccagttt

SEQ ID NO: 1399 - RNA, 20 nt, synthetic construct
  source 1..20: mol_type = other RNA
tatattacccagtttgggag

SEQ ID NO: 1400 - RNA, 20 nt, synthetic construct
  source 1..20: mol_type = other RNA
agttctgccactcccaaact

SEQ ID NO: 1401 - RNA, 20 nt, synthetic construct
  source 1..20: mol_type = other RNA
aagttctgccactcccaaac

SEQ ID NO: 1402 - RNA, 20 nt, synthetic construct
  source 1..20: mol_type = other RNA
ggttcttaatcaggtggaag

SEQ ID NO: 1403 - RNA, 20 nt, synthetic construct
  source 1..20: mol_type = other RNA
tacagtggttcttaatcagg

SEQ ID NO: 1404 - RNA, 20 nt, synthetic construct
  source 1..20: mol_type = other RNA
tgctacagtggttcttaatc

SEQ ID NO: 1405 - RNA, 20 nt, synthetic construct
  source 1..20: mol_type = other RNA
tgtagcagacgcagacttat

SEQ ID NO: 1406 - RNA, 20 nt, synthetic construct
  source 1..20: mol_type = other RNA
taagtctgcgtctgctacag

SEQ ID NO: 1407 - RNA, 20 nt, synthetic construct
  source 1..20: mol_type = other RNA
acgcagacttattggacact

SEQ ID NO: 1408 - RNA, 20 nt, synthetic construct
  source 1..20: mol_type = other RNA
cagacttattggacactagg

SEQ ID NO: 1409 - RNA, 20 nt, synthetic construct
  source 1..20: mol_type = other RNA
agacttattggacactaggc

SEQ ID NO: 1410 - RNA, 20 nt, synthetic construct
  source 1..20: mol_type = other RNA
cttattggacactaggcggg

SEQ ID NO: 1411 - RNA, 20 nt, synthetic construct
  source 1..20: mol_type = other RNA
aggccagctctgcagacagc

SEQ ID NO: 1412 - RNA, 20 nt, synthetic construct
  source 1..20: mol_type = other RNA
ctctgcagacagcaggtctc

SEQ ID NO: 1413 - RNA, 20 nt, synthetic construct
  source 1..20: mol_type = other RNA
agacctgctgtctgcagagc

SEQ ID NO: 1414 - RNA, 20 nt, synthetic construct
  source 1..20: mol_type = other RNA
gacagcaggtctcaggaaga

SEQ ID NO: 1415 - RNA, 20 nt, synthetic construct
  source 1..20: mol_type = other RNA
aggtctcaggaagacggtca

SEQ ID NO: 1416 - RNA, 20 nt, synthetic construct
  source 1..20: mol_type = other RNA
tcaggaagacggtcaaggca

SEQ ID NO: 1417 - RNA, 20 nt, synthetic construct
  source 1..20: mol_type = other RNA
ggctgctgatgatccgctta

SEQ ID NO: 1418 - RNA, 20 nt, synthetic construct
  source 1..20: mol_type = other RNA
gctgctgatgatccgcttat

SEQ ID NO: 1419 - RNA, 20 nt, synthetic construct
  source 1..20: mol_type = other RNA
acaataaacacacccataag

SEQ ID NO: 1420 - RNA, 20 nt, synthetic construct
  source 1..20: mol_type = other RNA
cttagcccatgttagatgcg

SEQ ID NO: 1421 - RNA, 20 nt, synthetic construct
  source 1..20: mol_type = other RNA
tggttcctcgcatctaacat

SEQ ID NO: 1422 - RNA, 20 nt, synthetic construct
  source 1..20: mol_type = other RNA
gtggttcctcgcatctaaca

SEQ ID NO: 1423 - RNA, 20 nt, synthetic construct
  source 1..20: mol_type = other RNA
gctgtcatttgcagtgtgag

SEQ ID NO: 1424 - RNA, 20 nt, synthetic construct
  source 1..20: mol_type = other RNA
acactgcaaatgacagctcc

SEQ ID NO: 1425 - RNA, 20 nt, synthetic construct
  source 1..20: mol_type = other RNA
tatgacactaagactgagcc

SEQ ID NO: 1426 - RNA, 20 nt, synthetic construct
  source 1..20: mol_type = other RNA
gtgtcatacttgcctttaac

SEQ ID NO: 1427 - RNA, 20 nt, synthetic construct
  source 1..20: mol_type = other RNA
gcaggggagttgccagttaa

SEQ ID NO: 1428 - RNA, 20 nt, synthetic construct
  source 1..20: mol_type = other RNA
tggcaactcccctgcaatac

SEQ ID NO: 1429 - RNA, 20 nt, synthetic construct
  source 1..20: mol_type = other RNA
ggcaactcccctgcaataca

SEQ ID NO: 1430 - RNA, 20 nt, synthetic construct
  source 1..20: mol_type = other RNA
gcctttcatggtgattaaga

SEQ ID NO: 1431 - RNA, 20 nt, synthetic construct
  source 1..20: mol_type = other RNA
cctttcatggtgattaagat

SEQ ID NO: 1432 - RNA, 20 nt, synthetic construct
  source 1..20: mol_type = other RNA
cccatcttaatcaccatgaa

SEQ ID NO: 1433 - RNA, 20 nt, synthetic construct
  source 1..20: mol_type = other RNA
attggttgttcacttaaata

SEQ ID NO: 1434 - RNA, 20 nt, synthetic construct
  source 1..20: mol_type = other RNA
ttggttgttcacttaaatat

SEQ ID NO: 1435 - RNA, 20 nt, synthetic construct
  source 1..20: mol_type = other RNA
cccctccccacccccaaatt

SEQ ID NO: 1436 - RNA, 20 nt, synthetic construct
  source 1..20: mol_type = other RNA
atttgggggtggggaggggt

SEQ ID NO: 1437 - RNA, 20 nt, synthetic construct
  source 1..20: mol_type = other RNA
aatttgggggtggggagggg

SEQ ID NO: 1438 - RNA, 20 nt, synthetic construct
  source 1..20: mol_type = other RNA
cctaatttgggggtggggag

SEQ ID NO: 1439 - RNA, 20 nt, synthetic construct
  source 1..20: mol_type = other RNA
ccctaatttgggggtgggga

SEQ ID NO: 1440 - RNA, 20 nt, synthetic construct
  source 1..20: mol_type = other RNA
tccctaatttgggggtgggg

SEQ ID NO: 1441 - RNA, 20 nt, synthetic construct
  source 1..20: mol_type = other RNA
ttctccctaatttgggggtg

SEQ ID NO: 1442 - RNA, 20 nt, synthetic construct
  source 1..20: mol_type = other RNA
tttctccctaatttgggggt

SEQ ID NO: 1443 - RNA, 20 nt, synthetic construct
  source 1..20: mol_type = other RNA
gtttctccctaatttggggg

SEQ ID NO: 1444 - RNA, 20 nt, synthetic construct
  source 1..20: mol_type = other RNA
ttagtttctccctaatttgg

SEQ ID NO: 1445 - RNA, 20 nt, synthetic construct
  source 1..20: mol_type = other RNA
cttagtttctccctaatttg

SEQ ID NO: 1446 - RNA, 20 nt, synthetic construct
  source 1..20: mol_type = other RNA
tcttagtttctccctaattt

SEQ ID NO: 1447 - RNA, 20 nt, synthetic construct
  source 1..20: mol_type = other RNA
ttcttagtttctccctaatt

SEQ ID NO: 1448 - RNA, 20 nt, synthetic construct
  source 1..20: mol_type = other RNA
agctttccttttgttgtttc

SEQ ID NO: 1449 - RNA, 20 nt, synthetic construct
  source 1..20: mol_type = other RNA
aaaatacctgaaacaacaaa

SEQ ID NO: 1450 - RNA, 20 nt, synthetic construct
  source 1..20: mol_type = other RNA
gttacgttacattgtccgcc

SEQ ID NO: 1451 - RNA, 20 nt, synthetic construct
  source 1..20: mol_type = other RNA
gttacattgtccgcctggtg

SEQ ID NO: 1452 - RNA, 20 nt, synthetic construct
  source 1..20: mol_type = other RNA
aatgcattctccacaccagg

SEQ ID NO: 1453 - RNA, 20 nt, synthetic construct
  source 1..20: mol_type = other RNA
ggtgtggagaatgcattgac

SEQ ID NO: 1454 - RNA, 20 nt, synthetic construct
  source 1..20: mol_type = other RNA
gtcaatgcattctccacacc

SEQ ID NO: 1455 - RNA, 20 nt, synthetic construct
  source 1..20: mol_type = other RNA
atgcattgacaggttctttg

SEQ ID NO: 1456 - RNA, 20 nt, synthetic construct
  source 1..20: mol_type = other RNA
aaaatgtctgcatggtatct

SEQ ID NO: 1457 - RNA, 20 nt, synthetic construct
  source 1..20: mol_type = other RNA
gaacaagcaaaatgtctgca

SEQ ID NO: 1458 - RNA, 20 nt, synthetic construct
  source 1..20: mol_type = other RNA
accaacaagacccagcaccg

SEQ ID NO: 1459 - RNA, 20 nt, synthetic construct
  source 1..20: mol_type = other RNA
accgcggtgctgggtcttgt

SEQ ID NO: 1460 - RNA, 20 nt, synthetic construct
  source 1..20: mol_type = other RNA
gacccagcaccgcggtctcc

SEQ ID NO: 1461 - RNA, 20 nt, synthetic construct
  source 1..20: mol_type = other RNA
caccaggagaccgcggtgct

SEQ ID NO: 1462 - RNA, 20 nt, synthetic construct
  source 1..20: mol_type = other RNA
gcaccaggagaccgcggtgc

SEQ ID NO: 1463 - RNA, 20 nt, synthetic construct
  source 1..20: mol_type = other RNA
ataatggcaccaggagaccg

SEQ ID NO: 1464 - RNA, 20 nt, synthetic construct
  source 1..20: mol_type = other RNA
ggctgcataataatggcacc

SEQ ID NO: 1465 - RNA, 20 nt, synthetic construct
  source 1..20: mol_type = other RNA
aaccgctggctgcataataa

SEQ ID NO: 1466 - RNA, 20 nt, synthetic construct
  source 1..20: mol_type = other RNA
tgcagccagcggttctcttg

SEQ ID NO: 1467 - RNA, 20 nt, synthetic construct
  source 1..20: mol_type = other RNA
agccagcggttctcttgtgg

SEQ ID NO: 1468 - RNA, 20 nt, synthetic construct
  source 1..20: mol_type = other RNA
gccagcggttctcttgtgga

SEQ ID NO: 1469 - RNA, 20 nt, synthetic construct
  source 1..20: mol_type = other RNA
ccagcggttctcttgtggag

SEQ ID NO: 1470 - RNA, 20 nt, synthetic construct
  source 1..20: mol_type = other RNA
cagcggttctcttgtggagg

SEQ ID NO: 1471 - RNA, 20 nt, synthetic construct
  source 1..20: mol_type = other RNA
ggttctcttgtggagggggc

SEQ ID NO: 1472 - RNA, 20 nt, synthetic construct
  source 1..20: mol_type = other RNA
cgtttcagaagacaccgagc

SEQ ID NO: 1473 - RNA, 20 nt, synthetic construct
  source 1..20: mol_type = other RNA
tcagaagacaccgagctgga

SEQ ID NO: 1474 - RNA, 20 nt, synthetic construct
  source 1..20: mol_type = other RNA
cagaagacaccgagctggat

SEQ ID NO: 1475 - RNA, 20 nt, synthetic construct
  source 1..20: mol_type = other RNA
aaaggtagtcccatccagct

SEQ ID NO: 1476 - RNA, 20 nt, synthetic construct
  source 1..20: mol_type = other RNA
ctgtgtggtgatgaacagaa

SEQ ID NO: 1477 - RNA, 20 nt, synthetic construct
  source 1..20: mol_type = other RNA
ccacacagcagaatttctaa

SEQ ID NO: 1478 - RNA, 20 nt, synthetic construct
  source 1..20: mol_type = other RNA
ccattagaaattctgctgtg

SEQ ID NO: 1479 - RNA, 20 nt, synthetic construct
  source 1..20: mol_type = other RNA
gaagtttgttgtgaatgtaa

SEQ ID NO: 1480 - RNA, 20 nt, synthetic construct
  source 1..20: mol_type = other RNA
gtttgttgtgaatgtaaagg

SEQ ID NO: 1481 - RNA, 20 nt, synthetic construct
  source 1..20: mol_type = other RNA
tttgttgtgaatgtaaagga

SEQ ID NO: 1482 - RNA, 20 nt, synthetic construct
  source 1..20: mol_type = other RNA
gctttttaatatacaaacca

SEQ ID NO: 1483 - RNA, 20 nt, synthetic construct
  source 1..20: mol_type = other RNA
atatacaaaccatggttttt

SEQ ID NO: 1484 - RNA, 20 nt, synthetic construct
  source 1..20: mol_type = other RNA
aaaccatggttttttggagc

SEQ ID NO: 1485 - RNA, 20 nt, synthetic construct
  source 1..20: mol_type = other RNA
aatcctgctccaaaaaacca

SEQ ID NO: 1486 - RNA, 20 nt, synthetic construct
  source 1..20: mol_type = other RNA
agcaggattttgtgtaagaa

SEQ ID NO: 1487 - RNA, 20 nt, synthetic construct
  source 1..20: mol_type = other RNA
tttccccctcaccttcaata

SEQ ID NO: 1488 - RNA, 20 nt, synthetic construct
  source 1..20: mol_type = other RNA
aaaccttattgaaggtgagg

SEQ ID NO: 1489 - RNA, 20 nt, synthetic construct
  source 1..20: mol_type = other RNA
aaaaccttattgaaggtgag

SEQ ID NO: 1490 - RNA, 20 nt, synthetic construct
  source 1..20: mol_type = other RNA
aaaaaccttattgaaggtga

SEQ ID NO: 1491 - RNA, 20 nt, synthetic construct
  source 1..20: mol_type = other RNA
gaaaaaccttattgaaggtg

SEQ ID NO: 1492 - RNA, 20 nt, synthetic construct
  source 1..20: mol_type = other RNA
ttcaataaggtttttcaaaa

SEQ ID NO: 1493 - RNA, 20 nt, synthetic construct
  source 1..20: mol_type = other RNA
tttttgaaaaaccttattga

SEQ ID NO: 1494 - RNA, 20 nt, synthetic construct
  source 1..20: mol_type = other RNA
aaggtttttcaaaaaggaaa

SEQ ID NO: 1495 - RNA, 20 nt, synthetic construct
  source 1..20: mol_type = other RNA
tacaaaagttattcacaaat

SEQ ID NO: 1496 - RNA, 20 nt, synthetic construct
  source 1..20: mol_type = other RNA
attaaaattttaagaaccta

SEQ ID NO: 1497 - RNA, 20 nt, synthetic construct
  source 1..20: mol_type = other RNA
aacctacggcctattctcag

SEQ ID NO: 1498 - RNA, 20 nt, synthetic construct
  source 1..20: mol_type = other RNA
atcctctgagaataggccgt

SEQ ID NO: 1499 - RNA, 20 nt, synthetic construct
  source 1..20: mol_type = other RNA
ttacataatcctctgagaat

SEQ ID NO: 1500 - RNA, 20 nt, synthetic construct
  source 1..20: mol_type = other RNA
ggattatgtaacccctgcag

SEQ ID NO: 1501 - RNA, 20 nt, synthetic construct
  source 1..20: mol_type = other RNA
tggctcagtttccactgcag

SEQ ID NO: 1502 - RNA, 20 nt, synthetic construct
  source 1..20: mol_type = other RNA
ctggctcagtttccactgca

SEQ ID NO: 1503 - RNA, 20 nt, synthetic construct
  source 1..20: mol_type = other RNA
gctggctcagtttccactgc

SEQ ID NO: 1504 - RNA, 20 nt, synthetic construct
  source 1..20: mol_type = other RNA
aggcagctttttaagttagc

SEQ ID NO: 1505 - RNA, 20 nt, synthetic construct
  source 1..20: mol_type = other RNA
taatctctaaaaataaacta

SEQ ID NO: 1506 - RNA, 20 nt, synthetic construct
  source 1..20: mol_type = other RNA
agattacagaatttttaaac

SEQ ID NO: 1507 - RNA, 20 nt, synthetic construct
  source 1..20: mol_type = other RNA
gattacagaatttttaaaca

SEQ ID NO: 1508 - RNA, 20 nt, synthetic construct
  source 1..20: mol_type = other RNA
aggcaatagtagggaaggga

SEQ ID NO: 1509 - RNA, 20 nt, synthetic construct
  source 1..20: mol_type = other RNA
gaggcaatagtagggaaggg

SEQ ID NO: 1510 - RNA, 20 nt, synthetic construct
  source 1..20: mol_type = other RNA
agagaggcaatagtagggaa

SEQ ID NO: 1511 - RNA, 20 nt, synthetic construct
  source 1..20: mol_type = other RNA
cagagaggcaatagtaggga

SEQ ID NO: 1512 - RNA, 20 nt, synthetic construct
  source 1..20: mol_type = other RNA
aggtcagagaggcaatagta

SEQ ID NO: 1513 - RNA, 20 nt, synthetic construct
  source 1..20: mol_type = other RNA
aaggtcagagaggcaatagt

SEQ ID NO: 1514 - RNA, 20 nt, synthetic construct
  source 1..20: mol_type = other RNA
ataatttaaaaaggtcagag

SEQ ID NO: 1515 - RNA, 20 nt, synthetic construct
  source 1..20: mol_type = other RNA
gtattaaaaataatttaaaa

SEQ ID NO: 1516 - RNA, 20 nt, synthetic construct
  source 1..20: mol_type = other RNA
ccaaaagagttcttttgaaa

SEQ ID NO: 1517 - RNA, 20 nt, synthetic construct
  source 1..20: mol_type = other RNA
ccatttcaaaagaactcttt

SEQ ID NO: 1518 - RNA, 20 nt, synthetic construct
  source 1..20: mol_type = other RNA
ttgaaatggaactgattaaa

SEQ ID NO: 1519 - RNA, 20 nt, synthetic construct
  source 1..20: mol_type = other RNA
tgaaatggaactgattaaaa

SEQ ID NO: 1520 - RNA, 20 nt, synthetic construct
  source 1..20: mol_type = other RNA
ggaactgattaaaagggcag

SEQ ID NO: 1521 - RNA, 20 nt, synthetic construct
  source 1..20: mol_type = other RNA
gaactgattaaaagggcaga

SEQ ID NO: 1522 - RNA, 20 nt, synthetic construct
  source 1..20: mol_type = other RNA
actggtatatcaatgcaggc

SEQ ID NO: 1523 - RNA, 20 nt, synthetic construct
  source 1..20: mol_type = other RNA
tgggactggtatatcaatgc

SEQ ID NO: 1524 - RNA, 20 nt, synthetic construct
  source 1..20: mol_type = other RNA
taaatatttacaaatgggac

SEQ ID NO: 1525 - RNA, 20 nt, synthetic construct
  source 1..20: mol_type = other RNA
gtacgtaaatatttacaaat

SEQ ID NO: 1526 - RNA, 20 nt, synthetic construct
  source 1..20: mol_type = other RNA
ggtacgtaaatatttacaaa

SEQ ID NO: 1527 - RNA, 20 nt, synthetic construct
  source 1..20: mol_type = other RNA
tataaattcagttgcatctg

SEQ ID NO: 1528 - RNA, 20 nt, synthetic construct
  source 1..20: mol_type = other RNA
agatgcaactgaatttataa

SEQ ID NO: 1529 - RNA, 20 nt, synthetic construct
  source 1..20: mol_type = other RNA
ttgcatcacaaaaagtgatg

SEQ ID NO: 1530 - RNA, 20 nt, synthetic construct
  source 1..20: mol_type = other RNA
tttgtgatgcaactccagtc

SEQ ID NO: 1531 - RNA, 20 nt, synthetic construct
  source 1..20: mol_type = other RNA
ctatgcatctgagtccagac

SEQ ID NO: 1532 - RNA, 20 nt, synthetic construct
  source 1..20: mol_type = other RNA
tggactcagatgcatagatt

SEQ ID NO: 1533 - RNA, 20 nt, synthetic construct
  source 1..20: mol_type = other RNA
actttatcatgaaaatacac

SEQ ID NO: 1534 - RNA, 20 nt, synthetic construct
  source 1..20: mol_type = other RNA
gctcgaactgtgcaagatac

SEQ ID NO: 1535 - RNA, 20 nt, synthetic construct
  source 1..20: mol_type = other RNA
tcgagcgatctgttattaac

SEQ ID NO: 1536 - RNA, 20 nt, synthetic construct
  source 1..20: mol_type = other RNA
cgagcgatctgttattaact

SEQ ID NO: 1537 - RNA, 20 nt, synthetic construct
  source 1..20: mol_type = other RNA
gttattaactgggaagcatt

SEQ ID NO: 1538 - RNA, 20 nt, synthetic construct
  source 1..20: mol_type = other RNA
aactgggaagcatttggtgt

SEQ ID NO: 1539 - RNA, 20 nt, synthetic construct
  source 1..20: mol_type = other RNA
catttcgacgagcatgttat

SEQ ID NO: 1540 - RNA, 20 nt, synthetic construct
  source 1..20: mol_type = other RNA
atttcgacgagcatgttatt

SEQ ID NO: 1541 - RNA, 20 nt, synthetic construct
  source 1..20: mol_type = other RNA
caataacatgctcgtcgaaa

SEQ ID NO: 1542 - RNA, 20 nt, synthetic construct
  source 1..20: mol_type = other RNA
tattgggaagtattctgaag

SEQ ID NO: 1543 - RNA, 20 nt, synthetic construct
  source 1..20: mol_type = other RNA
gctacgcccctttgtgctgc

SEQ ID NO: 1544 - RNA, 20 nt, synthetic construct
  source 1..20: mol_type = other RNA
ctttgtgctgctggcttttc

SEQ ID NO: 1545 - RNA, 20 nt, synthetic construct
  source 1..20: mol_type = other RNA
gaaaagccagcagcacaaag

SEQ ID NO: 1546 - RNA, 20 nt, synthetic construct
  source 1..20: mol_type = other RNA
agaaaagccagcagcacaaa

SEQ ID NO: 1547 - RNA, 20 nt, synthetic construct
  source 1..20: mol_type = other RNA
cagaaaagccagcagcacaa

SEQ ID NO: 1548 - RNA, 20 nt, synthetic construct
  source 1..20: mol_type = other RNA
ctgctggcttttctggttgc

SEQ ID NO: 1549 - RNA, 20 nt, synthetic construct
  source 1..20: mol_type = other RNA
tctggttgcaggctttccca

SEQ ID NO: 1550 - RNA, 20 nt, synthetic construct
  source 1..20: mol_type = other RNA
gcaggctttcccatggtcac

SEQ ID NO: 1551 - RNA, 20 nt, synthetic construct
  source 1..20: mol_type = other RNA
acagtgcatcctgtgaccat

SEQ ID NO: 1552 - RNA, 20 nt, synthetic construct
  source 1..20: mol_type = other RNA
gacagtgcatcctgtgacca

SEQ ID NO: 1553 - RNA, 20 nt, synthetic construct
  source 1..20: mol_type = other RNA
caggatgcactgtcagcatc

SEQ ID NO: 1554 - RNA, 20 nt, synthetic construct
  source 1..20: mol_type = other RNA
ctgtcagcatcaggtcccag

SEQ ID NO: 1555 - RNA, 20 nt, synthetic construct
  source 1..20: mol_type = other RNA
tgtcagcatcaggtcccaga

SEQ ID NO: 1556 - RNA, 20 nt, synthetic construct
  source 1..20: mol_type = other RNA
aatggacacggtggccctct

SEQ ID NO: 1557 - RNA, 20 nt, synthetic construct
  source 1..20: mol_type = other RNA
taatggacacggtggccctc

SEQ ID NO: 1558 - RNA, 20 nt, synthetic construct
  source 1..20: mol_type = other RNA
ctctgctgtaatggacacgg

SEQ ID NO: 1559 - RNA, 20 nt, synthetic construct
  source 1..20: mol_type = other RNA
ggactctgctgtaatggaca

SEQ ID NO: 1560 - RNA, 20 nt, synthetic construct
  source 1..20: mol_type = other RNA
gcagctggactctgctgtaa

SEQ ID NO: 1561 - RNA, 20 nt, synthetic construct
  source 1..20: mol_type = other RNA
cgtgagctggatgctgcagc

SEQ ID NO: 1562 - RNA, 20 nt, synthetic construct
  source 1..20: mol_type = other RNA
gcatccagctcacgccctca

SEQ ID NO: 1563 - RNA, 20 nt, synthetic construct
  source 1..20: mol_type = other RNA
catccagctcacgccctcat

SEQ ID NO: 1564 - RNA, 20 nt, synthetic construct
  source 1..20: mol_type = other RNA
gctcacgccctcatgggaat

SEQ ID NO: 1565 - RNA, 20 nt, synthetic construct
  source 1..20: mol_type = other RNA
attcccatgagggcgtgagc

SEQ ID NO: 1566 - RNA, 20 nt, synthetic construct
  source 1..20: mol_type = other RNA
gccctcatgggaattggcac

SEQ ID NO: 1567 - RNA, 20 nt, synthetic construct
  source 1..20: mol_type = other RNA
catgggaattggcacaggcc

SEQ ID NO: 1568 - RNA, 20 nt, synthetic construct
  source 1..20: mol_type = other RNA
atgggaattggcacaggcct

SEQ ID NO: 1569 - RNA, 20 nt, synthetic construct
  source 1..20: mol_type = other RNA
tgggaattggcacaggcctg

SEQ ID NO: 1570 - RNA, 20 nt, synthetic construct
  source 1..20: mol_type = other RNA
aattggcacaggcctggggc

SEQ ID NO: 1571 - RNA, 20 nt, synthetic construct
  source 1..20: mol_type = other RNA
attggcacaggcctggggca

SEQ ID NO: 1572 - RNA, 20 nt, synthetic construct
  source 1..20: mol_type = other RNA
gcctggggcagggcttctga

SEQ ID NO: 1573 - RNA, 20 nt, synthetic construct
  source 1..20: mol_type = other RNA
gccatcagaagccctgcccc

SEQ ID NO: 1574 - RNA, 20 nt, synthetic construct
  source 1..20: mol_type = other RNA
gcttctgatggccatttgct

SEQ ID NO: 1575 - RNA, 20 nt, synthetic construct
  source 1..20: mol_type = other RNA
aatgcaggaggccaagcaaa

SEQ ID NO: 1576 - RNA, 20 nt, synthetic construct
  source 1..20: mol_type = other RNA
gagttggactaaaatgcagg

SEQ ID NO: 1577 - RNA, 20 nt, synthetic construct
  source 1..20: mol_type = other RNA
tgtgagttggactaaaatgc

SEQ ID NO: 1578 - RNA, 20 nt, synthetic construct
  source 1..20: mol_type = other RNA
gaagctagtggactgtgagt

SEQ ID NO: 1579 - RNA, 20 nt, synthetic construct
  source 1..20: mol_type = other RNA
atttaaaggagtgaagctag

SEQ ID NO: 1580 - RNA, 20 nt, synthetic construct
  source 1..20: mol_type = other RNA
ctttaaattcactttgaaac

SEQ ID NO: 1581 - RNA, 20 nt, synthetic construct
  source 1..20: mol_type = other RNA
ctgtttcaaagtgaatttaa

SEQ ID NO: 1582 - RNA, 20 nt, synthetic construct
  source 1..20: mol_type = other RNA
gtgctggtggaagtgggatg

SEQ ID NO: 1583 - RNA, 20 nt, synthetic construct
  source 1..20: mol_type = other RNA
tctatggtgctggtggaagt

SEQ ID NO: 1584 - RNA, 20 nt, synthetic construct
  source 1..20: mol_type = other RNA
ttctatggtgctggtggaag

SEQ ID NO: 1585 - RNA, 20 nt, synthetic construct
  source 1..20: mol_type = other RNA
ttattcttctatggtgctgg

SEQ ID NO: 1586 - RNA, 20 nt, synthetic construct
  source 1..20: mol_type = other RNA
gcaccatagaagaataattc

SEQ ID NO: 1587 - RNA, 20 nt, synthetic construct
  source 1..20: mol_type = other RNA
caccatagaagaataattct

SEQ ID NO: 1588 - RNA, 20 nt, synthetic construct
  source 1..20: mol_type = other RNA
gaattattcttctatggtgc

SEQ ID NO: 1589 - RNA, 20 nt, synthetic construct
  source 1..20: mol_type = other RNA
tgcccagaattattcttcta

SEQ ID NO: 1590 - RNA, 20 nt, synthetic construct
  source 1..20: mol_type = other RNA
ctgttttttttcatttttcc

SEQ ID NO: 1591 - RNA, 20 nt, synthetic construct
  source 1..20: mol_type = other RNA
tttcatttttccaggacagt

SEQ ID NO: 1592 - RNA, 20 nt, synthetic construct
  source 1..20: mol_type = other RNA
caggacagttggatattgtc

SEQ ID NO: 1593 - RNA, 20 nt, synthetic construct
  source 1..20: mol_type = other RNA
ctgacaatatccaactgtcc

SEQ ID NO: 1594 - RNA, 20 nt, synthetic construct
  source 1..20: mol_type = other RNA
tacatggctggggtcacaag

SEQ ID NO: 1595 - RNA, 20 nt, synthetic construct
  source 1..20: mol_type = other RNA
gtgaccccagccatgtagtg

SEQ ID NO: 1596 - RNA, 20 nt, synthetic construct
  source 1..20: mol_type = other RNA
tgaccccagccatgtagtga

SEQ ID NO: 1597 - RNA, 20 nt, synthetic construct
  source 1..20: mol_type = other RNA
gcaccctcactacatggctg

SEQ ID NO: 1598 - RNA, 20 nt, synthetic construct
  source 1..20: mol_type = other RNA
agcaccctcactacatggct

SEQ ID NO: 1599 - RNA, 20 nt, synthetic construct
  source 1..20: mol_type = other RNA
gagcaccctcactacatggc

SEQ ID NO: 1600 - RNA, 20 nt, synthetic construct
  source 1..20: mol_type = other RNA
gaaagagcaccctcactaca

SEQ ID NO: 1601 - RNA, 20 nt, synthetic construct
  source 1..20: mol_type = other RNA
cctgctccttatgagtgcag

SEQ ID NO: 1602 - RNA, 20 nt, synthetic construct
  source 1..20: mol_type = other RNA
ctccttatgagtgcagtgga

SEQ ID NO: 1603 - RNA, 20 nt, synthetic construct
  source 1..20: mol_type = other RNA
ccactgcactcataaggagc

SEQ ID NO: 1604 - RNA, 20 nt, synthetic construct
  source 1..20: mol_type = other RNA
ttccttccactgcactcata

SEQ ID NO: 1605 - RNA, 20 nt, synthetic construct
  source 1..20: mol_type = other RNA
agtggaaggaagccacacac

SEQ ID NO: 1606 - RNA, 20 nt, synthetic construct
  source 1..20: mol_type = other RNA
acactggtcagtcatttcag

SEQ ID NO: 1607 - RNA, 20 nt, synthetic construct
  source 1..20: mol_type = other RNA
tgaaatgactgaccagtgtg

SEQ ID NO: 1608 - RNA, 20 nt, synthetic construct
  source 1..20: mol_type = other RNA
ttcagaggcagcagatgccc

SEQ ID NO: 1609 - RNA, 20 nt, synthetic construct
  source 1..20: mol_type = other RNA
tcagaggcagcagatgccca

SEQ ID NO: 1610 - RNA, 20 nt, synthetic construct
  source 1..20: mol_type = other RNA
gggagacccaagaaagagtc

SEQ ID NO: 1611 - RNA, 20 nt, synthetic construct
  source 1..20: mol_type = other RNA
actctttcttgggtctccct

SEQ ID NO: 1612 - RNA, 20 nt, synthetic construct
  source 1..20: mol_type = other RNA
gactctttcttgggtctccc

SEQ ID NO: 1613 - RNA, 20 nt, synthetic construct
  source 1..20: mol_type = other RNA
acccaagaaagagtcaggtt

SEQ ID NO: 1614 - RNA, 20 nt, synthetic construct
  source 1..20: mol_type = other RNA
cccaagaaagagtcaggtta

SEQ ID NO: 1615 - RNA, 20 nt, synthetic construct
  source 1..20: mol_type = other RNA
ccctaacctgactctttctt

SEQ ID NO: 1616 - RNA, 20 nt, synthetic construct
  source 1..20: mol_type = other RNA
tccctaacctgactctttct

SEQ ID NO: 1617 - RNA, 20 nt, synthetic construct
  source 1..20: mol_type = other RNA
gttagggagcagtgaaagtg

SEQ ID NO: 1618 - RNA, 20 nt, synthetic construct
  source 1..20: mol_type = other RNA
agggagcagtgaaagtgagg

SEQ ID NO: 1619 - RNA, 20 nt, synthetic construct
  source 1..20: mol_type = other RNA
gggagcagtgaaagtgagga

SEQ ID NO: 1620 - RNA, 20 nt, synthetic construct
  source 1..20: mol_type = other RNA
ttttaaaagttgtttaacga

SEQ ID NO: 1621 - RNA, 20 nt, synthetic construct
  source 1..20: mol_type = other RNA
tcgggcaaaacactagttgg

SEQ ID NO: 1622 - RNA, 20 nt, synthetic construct
  source 1..20: mol_type = other RNA
ctatcgggcaaaacactagt

SEQ ID NO: 1623 - RNA, 20 nt, synthetic construct
  source 1..20: mol_type = other RNA
aacatgctggctcttctatc

SEQ ID NO: 1624 - RNA, 20 nt, synthetic construct
  source 1..20: mol_type = other RNA
gaacatgctggctcttctat

SEQ ID NO: 1625 - RNA, 20 nt, synthetic construct
  source 1..20: mol_type = other RNA
tttaaataacgtgaacatgc

SEQ ID NO: 1626 - RNA, 20 nt, synthetic construct
  source 1..20: mol_type = other RNA
ttcacgttatttaaattagg

SEQ ID NO: 1627 - RNA, 20 nt, synthetic construct
  source 1..20: mol_type = other RNA
gcatattcactttttccttt

SEQ ID NO: 1628 - RNA, 20 nt, synthetic construct
  source 1..20: mol_type = other RNA
ttgaaatcatctctacctaa

SEQ ID NO: 1629 - RNA, 20 nt, synthetic construct
  source 1..20: mol_type = other RNA
ttttttaaagtaagagtatt

SEQ ID NO: 1630 - RNA, 20 nt, synthetic construct
  source 1..20: mol_type = other RNA
cctttccccaagaatctcct

SEQ ID NO: 1631 - RNA, 20 nt, synthetic construct
  source 1..20: mol_type = other RNA
ctttccccaagaatctcctt

SEQ ID NO: 1632 - RNA, 20 nt, synthetic construct
  source 1..20: mol_type = other RNA
ccaaggagattcttggggaa

SEQ ID NO: 1633 - RNA, 20 nt, synthetic construct
  source 1..20: mol_type = other RNA
aagtcccaaggagattcttg

SEQ ID NO: 1634 - RNA, 20 nt, synthetic construct
  source 1..20: mol_type = other RNA
aaagtcccaaggagattctt

SEQ ID NO: 1635 - RNA, 20 nt, synthetic construct
  source 1..20: mol_type = other RNA
caaagtcccaaggagattct

SEQ ID NO: 1636 - RNA, 20 nt, synthetic construct
  source 1..20: mol_type = other RNA
aaaaataagtcaaagtccca

SEQ ID NO: 1637 - RNA, 20 nt, synthetic construct
  source 1..20: mol_type = other RNA
acttatttttaaagctgtgt

SEQ ID NO: 1638 - RNA, 20 nt, synthetic construct
  source 1..20: mol_type = other RNA
ctgatgtgtctcgagcccat

SEQ ID NO: 1639 - RNA, 20 nt, synthetic construct
  source 1..20: mol_type = other RNA
aatgggctcgagacacatca

SEQ ID NO: 1640 - RNA, 20 nt, synthetic construct
  source 1..20: mol_type = other RNA
caatgggctcgagacacatc

SEQ ID NO: 1641 - RNA, 20 nt, synthetic construct
  source 1..20: mol_type = other RNA
gtgtctcgagcccattggta

SEQ ID NO: 1642 - RNA, 20 nt, synthetic construct
  source 1..20: mol_type = other RNA
ctttgtatgaccctaccaat

SEQ ID NO: 1643 - RNA, 20 nt, synthetic construct
  source 1..20: mol_type = other RNA
gctttgtatgaccctaccaa

SEQ ID NO: 1644 - RNA, 20 nt, synthetic construct
  source 1..20: mol_type = other RNA
gtagggtcatacaaagccca

SEQ ID NO: 1645 - RNA, 20 nt, synthetic construct
  source 1..20: mol_type = other RNA
aagcccacggttacaagcag

SEQ ID NO: 1646 - RNA, 20 nt, synthetic construct
  source 1..20: mol_type = other RNA
ccacggttacaagcagtggt

SEQ ID NO: 1647 - RNA, 20 nt, synthetic construct
  source 1..20: mol_type = other RNA
ctaccactgcttgtaaccgt

SEQ ID NO: 1648 - RNA, 20 nt, synthetic construct
  source 1..20: mol_type = other RNA
cctaccactgcttgtaaccg

SEQ ID NO: 1649 - RNA, 20 nt, synthetic construct
  source 1..20: mol_type = other RNA
cagtggtaggattgcagccg

SEQ ID NO: 1650 - RNA, 20 nt, synthetic construct
  source 1..20: mol_type = other RNA
agtggtaggattgcagccgt

SEQ ID NO: 1651 - RNA, 20 nt, synthetic construct
  source 1..20: mol_type = other RNA
gattgcagccgtgggcctgc

SEQ ID NO: 1652 - RNA, 20 nt, synthetic construct
  source 1..20: mol_type = other RNA
gtgtgtgtccagcaggccca

SEQ ID NO: 1653 - RNA, 20 nt, synthetic construct
  source 1..20: mol_type = other RNA
ggtgtatgtgtgtgtccagc

SEQ ID NO: 1654 - RNA, 20 nt, synthetic construct
  source 1..20: mol_type = other RNA
acatacaccaaagatgtatt

SEQ ID NO: 1655 - RNA, 20 nt, synthetic construct
  source 1..20: mol_type = other RNA
accaaagatgtatttggatc

SEQ ID NO: 1656 - RNA, 20 nt, synthetic construct
  source 1..20: mol_type = other RNA
ccaaagatgtatttggatct

SEQ ID NO: 1657 - RNA, 20 nt, synthetic construct
  source 1..20: mol_type = other RNA
cccagatccaaatacatctt

SEQ ID NO: 1658 - RNA, 20 nt, synthetic construct
  source 1..20: mol_type = other RNA
ggatctgggcaccccctccc

SEQ ID NO: 1659 - RNA, 20 nt, synthetic construct
  source 1..20: mol_type = other RNA
agtacagggatcctgggagg

SEQ ID NO: 1660 - RNA, 20 nt, synthetic construct
  source 1..20: mol_type = other RNA
gagtacagggatcctgggag

SEQ ID NO: 1661 - RNA, 20 nt, synthetic construct
  source 1..20: mol_type = other RNA
tgagtacagggatcctggga

SEQ ID NO: 1662 - RNA, 20 nt, synthetic construct
  source 1..20: mol_type = other RNA
gtgagtacagggatcctggg

SEQ ID NO: 1663 - RNA, 20 nt, synthetic construct
  source 1..20: mol_type = other RNA
cacgtgagtacagggatcct

SEQ ID NO: 1664 - RNA, 20 nt, synthetic construct
  source 1..20: mol_type = other RNA
gcacgtgagtacagggatcc

SEQ ID NO: 1665 - RNA, 20 nt, synthetic construct
  source 1..20: mol_type = other RNA
gagactggcacgtgagtaca

SEQ ID NO: 1666 - RNA, 20 nt, synthetic construct
  source 1..20: mol_type = other RNA
ggagactggcacgtgagtac

SEQ ID NO: 1667 - RNA, 20 nt, synthetic construct
  source 1..20: mol_type = other RNA
aagtgctctagtcaggagac

SEQ ID NO: 1668 - RNA, 20 nt, synthetic construct
  source 1..20: mol_type = other RNA
cagagtaaagtgctctagtc

SEQ ID NO: 1669 - RNA, 20 nt, synthetic construct
  source 1..20: mol_type = other RNA
ttcctcagccctgcagcccc

SEQ ID NO: 1670 - RNA, 20 nt, synthetic construct
  source 1..20: mol_type = other RNA
tcctcagccctgcagcccct

SEQ ID NO: 1671 - RNA, 20 nt, synthetic construct
  source 1..20: mol_type = other RNA
tcccaggggctgcagggctg

SEQ ID NO: 1672 - RNA, 20 nt, synthetic construct
  source 1..20: mol_type = other RNA
cagcccctgggagcacacac

SEQ ID NO: 1673 - RNA, 20 nt, synthetic construct
  source 1..20: mol_type = other RNA
agcccctgggagcacacact

SEQ ID NO: 1674 - RNA, 20 nt, synthetic construct
  source 1..20: mol_type = other RNA
cacccagtgtgtgctcccag

SEQ ID NO: 1675 - RNA, 20 nt, synthetic construct
  source 1..20: mol_type = other RNA
gcacccagtgtgtgctccca

SEQ ID NO: 1676 - RNA, 20 nt, synthetic construct
  source 1..20: mol_type = other RNA
tgcacccagtgtgtgctccc

SEQ ID NO: 1677 - RNA, 20 nt, synthetic construct
  source 1..20: mol_type = other RNA
gcacacactgggtgcagccc

SEQ ID NO: 1678 - RNA, 20 nt, synthetic construct
  source 1..20: mol_type = other RNA
cacacactgggtgcagccct

SEQ ID NO: 1679 - RNA, 20 nt, synthetic construct
  source 1..20: mol_type = other RNA
actgggtgcagccctgggcc

SEQ ID NO: 1680 - RNA, 20 nt, synthetic construct
  source 1..20: mol_type = other RNA
gtgcagccctgggccaggca

SEQ ID NO: 1681 - RNA, 20 nt, synthetic construct
  source 1..20: mol_type = other RNA
tgcagccctgggccaggcac

SEQ ID NO: 1682 - RNA, 20 nt, synthetic construct
  source 1..20: mol_type = other RNA
agccctgggccaggcacggg

SEQ ID NO: 1683 - RNA, 20 nt, synthetic construct
  source 1..20: mol_type = other RNA
ggcctcccgtgcctggccca

SEQ ID NO: 1684 - RNA, 20 nt, synthetic construct
  source 1..20: mol_type = other RNA
gggcctcccgtgcctggccc

SEQ ID NO: 1685 - RNA, 20 nt, synthetic construct
  source 1..20: mol_type = other RNA
agggcagggcctcccgtgcc

SEQ ID NO: 1686 - RNA, 20 nt, synthetic construct
  source 1..20: mol_type = other RNA
ggccctgccctgtgctgccc

SEQ ID NO: 1687 - RNA, 20 nt, synthetic construct
  source 1..20: mol_type = other RNA
gccctgccctgtgctgccca

SEQ ID NO: 1688 - RNA, 20 nt, synthetic construct
  source 1..20: mol_type = other RNA
ccctgccctgtgctgcccag

SEQ ID NO: 1689 - RNA, 20 nt, synthetic construct
  source 1..20: mol_type = other RNA
cccctgggcagcacagggca

SEQ ID NO: 1690 - RNA, 20 nt, synthetic construct
  source 1..20: mol_type = other RNA
gcccctgggcagcacagggc

SEQ ID NO: 1691 - RNA, 20 nt, synthetic construct
  source 1..20: mol_type = other RNA
cacagcccctgggcagcaca

SEQ ID NO: 1692 - RNA, 20 nt, synthetic construct
  source 1..20: mol_type = other RNA
acacagcccctgggcagcac

SEQ ID NO: 1693 - RNA, 20 nt, synthetic construct
  source 1..20: mol_type = other RNA
atgtggtgcacacagcccct

SEQ ID NO: 1694 - RNA, 20 nt, synthetic construct
  source 1..20: mol_type = other RNA
catgtggtgcacacagcccc

SEQ ID NO: 1695 - RNA, 20 nt, synthetic construct
  source 1..20: mol_type = other RNA
cacatgagcacatttccctc

SEQ ID NO: 1696 - RNA, 20 nt, synthetic construct
  source 1..20: mol_type = other RNA
cagagggaaatgtgctcatg

SEQ ID NO: 1697 - RNA, 20 nt, synthetic construct
  source 1..20: mol_type = other RNA
gagcacatttccctctggcc

SEQ ID NO: 1698 - RNA, 20 nt, synthetic construct
  source 1..20: mol_type = other RNA
cacatttccctctggcctgg

SEQ ID NO: 1699 - RNA, 20 nt, synthetic construct
  source 1..20: mol_type = other RNA
cctctggcctggcggcctcc

SEQ ID NO: 1700 - RNA, 20 nt, synthetic construct
  source 1..20: mol_type = other RNA
tggcctggcggcctccaggc

SEQ ID NO: 1701 - RNA, 20 nt, synthetic construct
  source 1..20: mol_type = other RNA
cctggaggccgccaggccag

SEQ ID NO: 1702 - RNA, 20 nt, synthetic construct
  source 1..20: mol_type = other RNA
ggcggcctccaggctggctg

SEQ ID NO: 1703 - RNA, 20 nt, synthetic construct
  source 1..20: mol_type = other RNA
cagccagcctggaggccgcc

SEQ ID NO: 1704 - RNA, 20 nt, synthetic construct
  source 1..20: mol_type = other RNA
tgtttccacagccagcctgg

SEQ ID NO: 1705 - RNA, 20 nt, synthetic construct
  source 1..20: mol_type = other RNA
aactgtttccacagccagcc

SEQ ID NO: 1706 - RNA, 20 nt, synthetic construct
  source 1..20: mol_type = other RNA
ggctgtggaaacagttcctg

SEQ ID NO: 1707 - RNA, 20 nt, synthetic construct
  source 1..20: mol_type = other RNA
atagaatctctaatttcctc

SEQ ID NO: 1708 - RNA, 20 nt, synthetic construct
  source 1..20: mol_type = other RNA
ttagagattctatgaattgt

SEQ ID NO: 1709 - RNA, 20 nt, synthetic construct
  source 1..20: mol_type = other RNA
ttgtaggagtattaaagacc

SEQ ID NO: 1710 - RNA, 20 nt, synthetic construct
  source 1..20: mol_type = other RNA
agtattaaagaccaggctgt

SEQ ID NO: 1711 - RNA, 20 nt, synthetic construct
  source 1..20: mol_type = other RNA
aagttctggtgccaacagcc

SEQ ID NO: 1712 - RNA, 20 nt, synthetic construct
  source 1..20: mol_type = other RNA
ccagaacttaaagcgatgac

SEQ ID NO: 1713 - RNA, 20 nt, synthetic construct
  source 1..20: mol_type = other RNA
ccagtcatcgctttaagttc

SEQ ID NO: 1714 - RNA, 20 nt, synthetic construct
  source 1..20: mol_type = other RNA
gtctctgtactgtatgtatc

SEQ ID NO: 1715 - RNA, 20 nt, synthetic construct
  source 1..20: mol_type = other RNA
gaggcatactttctgcacag

SEQ ID NO: 1716 - RNA, 20 nt, synthetic construct
  source 1..20: mol_type = other RNA
tgcagaaagtatgcctcccg

SEQ ID NO: 1717 - RNA, 20 nt, synthetic construct
  source 1..20: mol_type = other RNA
gcagaaagtatgcctcccgt

SEQ ID NO: 1718 - RNA, 20 nt, synthetic construct
  source 1..20: mol_type = other RNA
taaaaacgtatacccacggg

SEQ ID NO: 1719 - RNA, 20 nt, synthetic construct
  source 1..20: mol_type = other RNA
aggtaaaaacgtatacccac

SEQ ID NO: 1720 - RNA, 20 nt, synthetic construct
  source 1..20: mol_type = other RNA
aaggtaaaaacgtataccca

SEQ ID NO: 1721 - RNA, 20 nt, synthetic construct
  source 1..20: mol_type = other RNA
acaaaaatgttttttaaaaa

SEQ ID NO: 1722 - RNA, 20 nt, synthetic construct
  source 1..20: mol_type = other RNA
aaataattaaatcccctttt

SEQ ID NO: 1723 - RNA, 20 nt, synthetic construct
  source 1..20: mol_type = other RNA
cctttttggaaacttactgc

SEQ ID NO: 1724 - RNA, 20 nt, synthetic construct
  source 1..20: mol_type = other RNA
tgcagtaagtttccaaaaag

SEQ ID NO: 1725 - RNA, 20 nt, synthetic construct
  source 1..20: mol_type = other RNA
ctgcagtaagtttccaaaaa

SEQ ID NO: 1726 - RNA, 20 nt, synthetic construct
  source 1..20: mol_type = other RNA
cctgcagtaagtttccaaaa

SEQ ID NO: 1727 - RNA, 20 nt, synthetic construct
  source 1..20: mol_type = other RNA
tgacaacctctccctatgtg

SEQ ID NO: 1728 - RNA, 20 nt, synthetic construct
  source 1..20: mol_type = other RNA
cacatagggagaggttgtca

SEQ ID NO: 1729 - RNA, 20 nt, synthetic construct
  source 1..20: mol_type = other RNA
tacaaacctcacatagggag

SEQ ID NO: 1730 - RNA, 20 nt, synthetic construct
  source 1..20: mol_type = other RNA
ctttttacaaacctcacata

SEQ ID NO: 1731 - RNA, 20 nt, synthetic construct
  source 1..20: mol_type = other RNA
actttttacaaacctcacat

SEQ ID NO: 1732 - RNA, 20 nt, synthetic construct
  source 1..20: mol_type = other RNA
gcgtttctgtgttaagtcac

SEQ ID NO: 1733 - RNA, 20 nt, synthetic construct
  source 1..20: mol_type = other RNA
cttcagatgcccttcccaac

SEQ ID NO: 1734 - RNA, 20 nt, synthetic construct
  source 1..20: mol_type = other RNA
atcaactaaccagttgggaa

SEQ ID NO: 1735 - RNA, 20 nt, synthetic construct
  source 1..20: mol_type = other RNA
gatcaactaaccagttggga

SEQ ID NO: 1736 - RNA, 20 nt, synthetic construct
  source 1..20: mol_type = other RNA
tcttgatcaactaaccagtt

SEQ ID NO: 1737 - RNA, 20 nt, synthetic construct
  source 1..20: mol_type = other RNA
ttcttgatcaactaaccagt

SEQ ID NO: 1738 - RNA, 20 nt, synthetic construct
  source 1..20: mol_type = other RNA
ggttagttgatcaagaattt

SEQ ID NO: 1739 - RNA, 20 nt, synthetic construct
  source 1..20: mol_type = other RNA
gttagttgatcaagaatttt

SEQ ID NO: 1740 - RNA, 20 nt, synthetic construct
  source 1..20: mol_type = other RNA
ttagttgatcaagaattttg

SEQ ID NO: 1741 - RNA, 20 nt, synthetic construct
  source 1..20: mol_type = other RNA
tagttgatcaagaattttgg

SEQ ID NO: 1742 - RNA, 20 nt, synthetic construct
  source 1..20: mol_type = other RNA
ttgatcaagaattttggggg

SEQ ID NO: 1743 - RNA, 20 nt, synthetic construct
  source 1..20: mol_type = other RNA
tgatcaagaattttgggggt

SEQ ID NO: 1744 - RNA, 20 nt, synthetic construct
  source 1..20: mol_type = other RNA
gatcaagaattttgggggtg

SEQ ID NO: 1745 - RNA, 20 nt, synthetic construct
  source 1..20: mol_type = other RNA
atcaagaattttgggggtgg

SEQ ID NO: 1746 - RNA, 20 nt, synthetic construct
  source 1..20: mol_type = other RNA
aattttgggggtgggggttg

SEQ ID NO: 1747 - RNA, 20 nt, synthetic construct
  source 1..20: mol_type = other RNA
ttctgattaaaaaaatatag

SEQ ID NO: 1748 - RNA, 20 nt, synthetic construct
  source 1..20: mol_type = other RNA
actatatttttttaatcaga

SEQ ID NO: 1749 - RNA, 20 nt, synthetic construct
  source 1..20: mol_type = other RNA
tatacattaagaaggggaaa

SEQ ID NO: 1750 - RNA, 20 nt, synthetic construct
  source 1..20: mol_type = other RNA
acaatatatacattaagaag

SEQ ID NO: 1751 - RNA, 20 nt, synthetic construct
  source 1..20: mol_type = other RNA
cacaatatatacattaagaa

SEQ ID NO: 1752 - RNA, 20 nt, synthetic construct
  source 1..20: mol_type = other RNA
tcacaatatatacattaaga

SEQ ID NO: 1753 - RNA, 20 nt, synthetic construct
  source 1..20: mol_type = other RNA
tgagtatttattagattcgt

SEQ ID NO: 1754 - RNA, 20 nt, synthetic construct
  source 1..20: mol_type = other RNA
cacaattgcacacagacatt

SEQ ID NO: 1755 - RNA, 20 nt, synthetic construct
  source 1..20: mol_type = other RNA
tacaaaattttacaaggtaa

SEQ ID NO: 1756 - RNA, 20 nt, synthetic construct
  source 1..20: mol_type = other RNA
atgctgtacaaaattttaca

SEQ ID NO: 1757 - RNA, 20 nt, synthetic construct
  source 1..20: mol_type = other RNA
tctcaactttttcaaaatca

SEQ ID NO: 1758 - RNA, 20 nt, synthetic construct
  source 1..20: mol_type = other RNA
ttacagcattatgaaacagt

SEQ ID NO: 1759 - RNA, 20 nt, synthetic construct
  source 1..20: mol_type = other RNA
cggcaggggagtgggagaca

SEQ ID NO: 1760 - RNA, 20 nt, synthetic construct
  source 1..20: mol_type = other RNA
acggcaggggagtgggagac

SEQ ID NO: 1761 - RNA, 20 nt, synthetic construct
  source 1..20: mol_type = other RNA
tcatgggacggcaggggagt

SEQ ID NO: 1762 - RNA, 20 nt, synthetic construct
  source 1..20: mol_type = other RNA
ttcatgggacggcaggggag

SEQ ID NO: 1763 - RNA, 20 nt, synthetic construct
  source 1..20: mol_type = other RNA
ttaacttcatgggacggcag

SEQ ID NO: 1764 - RNA, 20 nt, synthetic construct
  source 1..20: mol_type = other RNA
gttaacttcatgggacggca

SEQ ID NO: 1765 - RNA, 20 nt, synthetic construct
  source 1..20: mol_type = other RNA
agttaacttcatgggacggc

SEQ ID NO: 1766 - RNA, 20 nt, synthetic construct
  source 1..20: mol_type = other RNA
caggagttaacttcatggga

SEQ ID NO: 1767 - RNA, 20 nt, synthetic construct
  source 1..20: mol_type = other RNA
ctctcaggagttaacttcat

SEQ ID NO: 1768 - RNA, 20 nt, synthetic construct
  source 1..20: mol_type = other RNA
actctcaggagttaacttca

SEQ ID NO: 1769 - RNA, 20 nt, synthetic construct
  source 1..20: mol_type = other RNA
agttaactcctgagagttgt

SEQ ID NO: 1770 - RNA, 20 nt, synthetic construct
  source 1..20: mol_type = other RNA
gttaactcctgagagttgtc

SEQ ID NO: 1771 - RNA, 20 nt, synthetic construct
  source 1..20: mol_type = other RNA
ttaactcctgagagttgtcg

SEQ ID NO: 1772 - RNA, 20 nt, synthetic construct
  source 1..20: mol_type = other RNA
taactcctgagagttgtcgg

SEQ ID NO: 1773 - RNA, 20 nt, synthetic construct
  source 1..20: mol_type = other RNA
tgagagttgtcgggggtgac

SEQ ID NO: 1774 - RNA, 20 nt, synthetic construct
  source 1..20: mol_type = other RNA
agtcacccccgacaactctc

SEQ ID NO: 1775 - RNA, 20 nt, synthetic construct
  source 1..20: mol_type = other RNA
agagctcattgcagaccacg

SEQ ID NO: 1776 - RNA, 20 nt, synthetic construct
  source 1..20: mol_type = other RNA
tgcagaccacgtggtcctcc

SEQ ID NO: 1777 - RNA, 20 nt, synthetic construct
  source 1..20: mol_type = other RNA
gcagaccacgtggtcctcca

SEQ ID NO: 1778 - RNA, 20 nt, synthetic construct
  source 1..20: mol_type = other RNA
gaccacgtggtcctccaggg

SEQ ID NO: 1779 - RNA, 20 nt, synthetic construct
  source 1..20: mol_type = other RNA
agccaccctggaggaccacg

SEQ ID NO: 1780 - RNA, 20 nt, synthetic construct
  source 1..20: mol_type = other RNA
ccagggtggctctccacctt

SEQ ID NO: 1781 - RNA, 20 nt, synthetic construct
  source 1..20: mol_type = other RNA
cagggtggctctccaccttc

SEQ ID NO: 1782 - RNA, 20 nt, synthetic construct
  source 1..20: mol_type = other RNA
aaggtggagagccaccctgg

SEQ ID NO: 1783 - RNA, 20 nt, synthetic construct
  source 1..20: mol_type = other RNA
ccgaaggtggagagccaccc

SEQ ID NO: 1784 - RNA, 20 nt, synthetic construct
  source 1..20: mol_type = other RNA
ggctctccaccttcgggtcc

SEQ ID NO: 1785 - RNA, 20 nt, synthetic construct
  source 1..20: mol_type = other RNA
gaaataccaggacccgaagg

SEQ ID NO: 1786 - RNA, 20 nt, synthetic construct
  source 1..20: mol_type = other RNA
ctggaaataccaggacccga

SEQ ID NO: 1787 - RNA, 20 nt, synthetic construct
  source 1..20: mol_type = other RNA
tcctggtatttccagtcaag

SEQ ID NO: 1788 - RNA, 20 nt, synthetic construct
  source 1..20: mol_type = other RNA
cctggtatttccagtcaagt

SEQ ID NO: 1789 - RNA, 20 nt, synthetic construct
  source 1..20: mol_type = other RNA
cccacttgactggaaatacc

SEQ ID NO: 1790 - RNA, 20 nt, synthetic construct
  source 1..20: mol_type = other RNA
gtcaagtgggtttcaattct

SEQ ID NO: 1791 - RNA, 20 nt, synthetic construct
  source 1..20: mol_type = other RNA
tcaagtgggtttcaattctt

SEQ ID NO: 1792 - RNA, 20 nt, synthetic construct
  source 1..20: mol_type = other RNA
agaattgaaacccacttgac

SEQ ID NO: 1793 - RNA, 20 nt, synthetic construct
  source 1..20: mol_type = other RNA
cacacacttcatcataaggg

SEQ ID NO: 1794 - RNA, 20 nt, synthetic construct
  source 1..20: mol_type = other RNA
aaacacacacttcatcataa

SEQ ID NO: 1795 - RNA, 20 nt, synthetic construct
  source 1..20: mol_type = other RNA
caaacacacacttcatcata

SEQ ID NO: 1796 - RNA, 20 nt, synthetic construct
  source 1..20: mol_type = other RNA
tgccagtgagaaactcagtc

SEQ ID NO: 1797 - RNA, 20 nt, synthetic construct
  source 1..20: mol_type = other RNA
agtgagaaactcagtctggc

SEQ ID NO: 1798 - RNA, 20 nt, synthetic construct
  source 1..20: mol_type = other RNA
tgccagactgagtttctcac

SEQ ID NO: 1799 - RNA, 20 nt, synthetic construct
  source 1..20: mol_type = other RNA
gaaggttgctgggtatttct

SEQ ID NO: 1800 - RNA, 20 nt, synthetic construct
  source 1..20: mol_type = other RNA
ggaacaaacagaaggttgct

SEQ ID NO: 1801 - RNA, 20 nt, synthetic construct
  source 1..20: mol_type = other RNA
tggaacaaacagaaggttgc

SEQ ID NO: 1802 - RNA, 20 nt, synthetic construct
  source 1..20: mol_type = other RNA
gttgctttggaacaaacaga

SEQ ID NO: 1803 - RNA, 20 nt, synthetic construct
  source 1..20: mol_type = other RNA
gcatgataagctagttgctt

SEQ ID NO: 1804 - RNA, 20 nt, synthetic construct
  source 1..20: mol_type = other RNA
aagcaaattttgctgactcc

SEQ ID NO: 1805 - RNA, 20 nt, synthetic construct
  source 1..20: mol_type = other RNA
tgactccaggctttatcttt

SEQ ID NO: 1806 - RNA, 20 nt, synthetic construct
  source 1..20: mol_type = other RNA
gttttcctaaagataaagcc

SEQ ID NO: 1807 - RNA, 20 nt, synthetic construct
  source 1..20: mol_type = other RNA
aaaaccaaagtattatcagc

SEQ ID NO: 1808 - RNA, 20 nt, synthetic construct
  source 1..20: mol_type = other RNA
accaaagtattatcagcagg

SEQ ID NO: 1809 - RNA, 20 nt, synthetic construct
  source 1..20: mol_type = other RNA
ccaaagtattatcagcaggt

SEQ ID NO: 1810 - RNA, 20 nt, synthetic construct
  source 1..20: mol_type = other RNA
cccacctgctgataatactt

SEQ ID NO: 1811 - RNA, 20 nt, synthetic construct
  source 1..20: mol_type = other RNA
ttctaaacgctgagttgtca

SEQ ID NO: 1812 - RNA, 20 nt, synthetic construct
  source 1..20: mol_type = other RNA
tttctaaacgctgagttgtc

SEQ ID NO: 1813 - RNA, 20 nt, synthetic construct
  source 1..20: mol_type = other RNA
ataaaatgtgccacttccag

SEQ ID NO: 1814 - RNA, 20 nt, synthetic construct
  source 1..20: mol_type = other RNA
caatgcagcacctctggaag

SEQ ID NO: 1815 - RNA, 20 nt, synthetic construct
  source 1..20: mol_type = other RNA
caactgcaatgcagcacctc

SEQ ID NO: 1816 - RNA, 20 nt, synthetic construct
  source 1..20: mol_type = other RNA
gtgctgcattgcagttgttc

SEQ ID NO: 1817 - RNA, 20 nt, synthetic construct
  source 1..20: mol_type = other RNA
tgctgcattgcagttgttca

SEQ ID NO: 1818 - RNA, 20 nt, synthetic construct
  source 1..20: mol_type = other RNA
cattgcagttgttcagggct

SEQ ID NO: 1819 - RNA, 20 nt, synthetic construct
  source 1..20: mol_type = other RNA
attgcagttgttcagggcta

SEQ ID NO: 1820 - RNA, 20 nt, synthetic construct
  source 1..20: mol_type = other RNA
agttgttcagggctagggcc

SEQ ID NO: 1821 - RNA, 20 nt, synthetic construct
  source 1..20: mol_type = other RNA
gttcagggctagggccaggc

SEQ ID NO: 1822 - RNA, 20 nt, synthetic construct
  source 1..20: mol_type = other RNA
ggccaggcaggacaagtgaa

SEQ ID NO: 1823 - RNA, 20 nt, synthetic construct
  source 1..20: mol_type = other RNA
gccaggcaggacaagtgaat

SEQ ID NO: 1824 - RNA, 20 nt, synthetic construct
  source 1..20: mol_type = other RNA
aggcaggacaagtgaatggg

SEQ ID NO: 1825 - RNA, 20 nt, synthetic construct
  source 1..20: mol_type = other RNA
ggcaggacaagtgaatgggt

SEQ ID NO: 1826 - RNA, 20 nt, synthetic construct
  source 1..20: mol_type = other RNA
acccattcacttgtcctgcc

SEQ ID NO: 1827 - RNA, 20 nt, synthetic construct
  source 1..20: mol_type = other RNA
gacaagtgaatgggtgggac

SEQ ID NO: 1828 - RNA, 20 nt, synthetic construct
  source 1..20: mol_type = other RNA
aagtgaatgggtgggacagg

SEQ ID NO: 1829 - RNA, 20 nt, synthetic construct
  source 1..20: mol_type = other RNA
ggacaggtggctcctgccta

SEQ ID NO: 1830 - RNA, 20 nt, synthetic construct
  source 1..20: mol_type = other RNA
tcctgcctaaggaccacctc

SEQ ID NO: 1831 - RNA, 20 nt, synthetic construct
  source 1..20: mol_type = other RNA
gcctgaggtggtccttaggc

SEQ ID NO: 1832 - RNA, 20 nt, synthetic construct
  source 1..20: mol_type = other RNA
agtggcctgaggtggtcctt

SEQ ID NO: 1833 - RNA, 20 nt, synthetic construct
  source 1..20: mol_type = other RNA
ctcaggccactaaccccttg

SEQ ID NO: 1834 - RNA, 20 nt, synthetic construct
  source 1..20: mol_type = other RNA
aaggggttagtggcctgagg

SEQ ID NO: 1835 - RNA, 20 nt, synthetic construct
  source 1..20: mol_type = other RNA
cacaaggggttagtggcctg

SEQ ID NO: 1836 - RNA, 20 nt, synthetic construct
  source 1..20: mol_type = other RNA
agttgtccacaaggggttag

SEQ ID NO: 1837 - RNA, 20 nt, synthetic construct
  source 1..20: mol_type = other RNA
tgtggacaactgtgagtagc

SEQ ID NO: 1838 - RNA, 20 nt, synthetic construct
  source 1..20: mol_type = other RNA
ctactcacagttgtccacaa

SEQ ID NO: 1839 - RNA, 20 nt, synthetic construct
  source 1..20: mol_type = other RNA
gctactcacagttgtccaca

SEQ ID NO: 1840 - RNA, 20 nt, synthetic construct
  source 1..20: mol_type = other RNA
ggaagttgcacagcaggtgg

SEQ ID NO: 1841 - RNA, 20 nt, synthetic construct
  source 1..20: mol_type = other RNA
aggaagttgcacagcaggtg

SEQ ID NO: 1842 - RNA, 20 nt, synthetic construct
  source 1..20: mol_type = other RNA
caggaagttgcacagcaggt

SEQ ID NO: 1843 - RNA, 20 nt, synthetic construct
  source 1..20: mol_type = other RNA
acaggaagttgcacagcagg

SEQ ID NO: 1844 - RNA, 20 nt, synthetic construct
  source 1..20: mol_type = other RNA
agcacaggaagttgcacagc

SEQ ID NO: 1845 - RNA, 20 nt, synthetic construct
  source 1..20: mol_type = other RNA
gtgcaacttcctgtgctttg

SEQ ID NO: 1846 - RNA, 20 nt, synthetic construct
  source 1..20: mol_type = other RNA
aacttcctgtgctttgaggt

SEQ ID NO: 1847 - RNA, 20 nt, synthetic construct
  source 1..20: mol_type = other RNA
ttagtccaacctcaaagcac

SEQ ID NO: 1848 - RNA, 20 nt, synthetic construct
  source 1..20: mol_type = other RNA
ggttggactaacttgtcttc

SEQ ID NO: 1849 - RNA, 20 nt, synthetic construct
  source 1..20: mol_type = other RNA
ctccccacgccccacccata

SEQ ID NO: 1850 - RNA, 20 nt, synthetic construct
  source 1..20: mol_type = other RNA
gtatgggtggggcgtgggga

SEQ ID NO: 1851 - RNA, 20 nt, synthetic construct
  source 1..20: mol_type = other RNA
cgtatgggtggggcgtgggg

SEQ ID NO: 1852 - RNA, 20 nt, synthetic construct
  source 1..20: mol_type = other RNA
gaccgtatgggtggggcgtg

SEQ ID NO: 1853 - RNA, 20 nt, synthetic construct
  source 1..20: mol_type = other RNA
tgaccgtatgggtggggcgt

SEQ ID NO: 1854 - RNA, 20 nt, synthetic construct
  source 1..20: mol_type = other RNA
gtgaccgtatgggtggggcg

SEQ ID NO: 1855 - RNA, 20 nt, synthetic construct
  source 1..20: mol_type = other RNA
acccatacggtcactgcatt

SEQ ID NO: 1856 - RNA, 20 nt, synthetic construct
  source 1..20: mol_type = other RNA
atgcagtgaccgtatgggtg

SEQ ID NO: 1857 - RNA, 20 nt, synthetic construct
  source 1..20: mol_type = other RNA
aatgcagtgaccgtatgggt

SEQ ID NO: 1858 - RNA, 20 nt, synthetic construct
  source 1..20: mol_type = other RNA
aaatgcagtgaccgtatggg

SEQ ID NO: 1859 - RNA, 20 nt, synthetic construct
  source 1..20: mol_type = other RNA
accaaatgcagtgaccgtat

SEQ ID NO: 1860 - RNA, 20 nt, synthetic construct
  source 1..20: mol_type = other RNA
gaccaaatgcagtgaccgta

SEQ ID NO: 1861 - RNA, 20 nt, synthetic construct
  source 1..20: mol_type = other RNA
tttggtcagcctgcttcttc

SEQ ID NO: 1862 - RNA, 20 nt, synthetic construct
  source 1..20: mol_type = other RNA
gggcatcgacctgaagaagc

SEQ ID NO: 1863 - RNA, 20 nt, synthetic construct
  source 1..20: mol_type = other RNA
gagatggagtatcagaagga

SEQ ID NO: 1864 - RNA, 20 nt, synthetic construct
  source 1..20: mol_type = other RNA
ggagatggagtatcagaagg

SEQ ID NO: 1865 - RNA, 20 nt, synthetic construct
  source 1..20: mol_type = other RNA
tctgatactccatctccttc

SEQ ID NO: 1866 - RNA, 20 nt, synthetic construct
  source 1..20: mol_type = other RNA
ctgatactccatctccttca

SEQ ID NO: 1867 - RNA, 20 nt, synthetic construct
  source 1..20: mol_type = other RNA
gaaggagatggagtatcaga

SEQ ID NO: 1868 - RNA, 20 nt, synthetic construct
  source 1..20: mol_type = other RNA
tactccatctccttcagggg

SEQ ID NO: 1869 - RNA, 20 nt, synthetic construct
  source 1..20: mol_type = other RNA
ccatctccttcaggggaggt

SEQ ID NO: 1870 - RNA, 20 nt, synthetic construct
  source 1..20: mol_type = other RNA
catctccttcaggggaggtt

SEQ ID NO: 1871 - RNA, 20 nt, synthetic construct
  source 1..20: mol_type = other RNA
atctccttcaggggaggttg

SEQ ID NO: 1872 - RNA, 20 nt, synthetic construct
  source 1..20: mol_type = other RNA
ccaacctcccctgaaggaga

SEQ ID NO: 1873 - RNA, 20 nt, synthetic construct
  source 1..20: mol_type = other RNA
aggggaggttggggccccac

SEQ ID NO: 1874 - RNA, 20 nt, synthetic construct
  source 1..20: mol_type = other RNA
aggttggggccccactggac

SEQ ID NO: 1875 - RNA, 20 nt, synthetic construct
  source 1..20: mol_type = other RNA
ggttggggccccactggact

SEQ ID NO: 1876 - RNA, 20 nt, synthetic construct
  source 1..20: mol_type = other RNA
tcttgacacccagtccagtg

SEQ ID NO: 1877 - RNA, 20 nt, synthetic construct
  source 1..20: mol_type = other RNA
atcttgacacccagtccagt

SEQ ID NO: 1878 - RNA, 20 nt, synthetic construct
  source 1..20: mol_type = other RNA
catcttgacacccagtccag

SEQ ID NO: 1879 - RNA, 20 nt, synthetic construct
  source 1..20: mol_type = other RNA
tgtcaagatgtgaaagctta

SEQ ID NO: 1880 - RNA, 20 nt, synthetic construct
  source 1..20: mol_type = other RNA
gtcaagatgtgaaagcttat

SEQ ID NO: 1881 - RNA, 20 nt, synthetic construct
  source 1..20: mol_type = other RNA
gaaagcttatgggagcttta

SEQ ID NO: 1882 - RNA, 20 nt, synthetic construct
  source 1..20: mol_type = other RNA
ggagctttaaggagacttca

SEQ ID NO: 1883 - RNA, 20 nt, synthetic construct
  source 1..20: mol_type = other RNA
gctttaaggagacttcatgg

SEQ ID NO: 1884 - RNA, 20 nt, synthetic construct
  source 1..20: mol_type = other RNA
acttcatggtggttccatgc

SEQ ID NO: 1885 - RNA, 20 nt, synthetic construct
  source 1..20: mol_type = other RNA
tcatggtggttccatgcagg

SEQ ID NO: 1886 - RNA, 20 nt, synthetic construct
  source 1..20: mol_type = other RNA
ggatggcagaaccacctgca

SEQ ID NO: 1887 - RNA, 20 nt, synthetic construct
  source 1..20: mol_type = other RNA
ccatccctgctgatttagcc

SEQ ID NO: 1888 - RNA, 20 nt, synthetic construct
  source 1..20: mol_type = other RNA
ccaggctaaatcagcaggga

SEQ ID NO: 1889 - RNA, 20 nt, synthetic construct
  source 1..20: mol_type = other RNA
ggcaccaggctaaatcagca

SEQ ID NO: 1890 - RNA, 20 nt, synthetic construct
  source 1..20: mol_type = other RNA
aggcaccaggctaaatcagc

SEQ ID NO: 1891 - RNA, 20 nt, synthetic construct
  source 1..20: mol_type = other RNA
agtggacacacacaggcacc

SEQ ID NO: 1892 - RNA, 20 nt, synthetic construct
  source 1..20: mol_type = other RNA
gtacgtgagtggacacacac

SEQ ID NO: 1893 - RNA, 20 nt, synthetic construct
  source 1..20: mol_type = other RNA
tgtgtccactcacgtacacg

SEQ ID NO: 1894 - RNA, 20 nt, synthetic construct
  source 1..20: mol_type = other RNA
gtgtccactcacgtacacgt

SEQ ID NO: 1895 - RNA, 20 nt, synthetic construct
  source 1..20: mol_type = other RNA
tgtccactcacgtacacgtg

SEQ ID NO: 1896 - RNA, 20 nt, synthetic construct
  source 1..20: mol_type = other RNA
ccactcacgtacacgtgggg

SEQ ID NO: 1897 - RNA, 20 nt, synthetic construct
  source 1..20: mol_type = other RNA
cactcacgtacacgtggggt

SEQ ID NO: 1898 - RNA, 20 nt, synthetic construct
  source 1..20: mol_type = other RNA
actcacgtacacgtggggtg

SEQ ID NO: 1899 - RNA, 20 nt, synthetic construct
  source 1..20: mol_type = other RNA
ctcacgtacacgtggggtgg

SEQ ID NO: 1900 - RNA, 20 nt, synthetic construct
  source 1..20: mol_type = other RNA
ccaccccacgtgtacgtgag

SEQ ID NO: 1901 - RNA, 20 nt, synthetic construct
  source 1..20: mol_type = other RNA
acagatgacgctaaatcagt

SEQ ID NO: 1902 - RNA, 20 nt, synthetic construct
  source 1..20: mol_type = other RNA
cagatgacgctaaatcagtt

SEQ ID NO: 1903 - RNA, 20 nt, synthetic construct
  source 1..20: mol_type = other RNA
agatgacgctaaatcagttg

SEQ ID NO: 1904 - RNA, 20 nt, synthetic construct
  source 1..20: mol_type = other RNA
gttacttaactgggagcttg

SEQ ID NO: 1905 - RNA, 20 nt, synthetic construct
  source 1..20: mol_type = other RNA
agtagtcaagttacttaact

SEQ ID NO: 1906 - RNA, 20 nt, synthetic construct
  source 1..20: mol_type = other RNA
aagtagtcaagttacttaac

SEQ ID NO: 1907 - RNA, 20 nt, synthetic construct
  source 1..20: mol_type = other RNA
gtaacttgactacttttatt

SEQ ID NO: 1908 - RNA, 20 nt, synthetic construct
  source 1..20: mol_type = other RNA
taacttgactacttttattt

SEQ ID NO: 1909 - RNA, 20 nt, synthetic construct
  source 1..20: mol_type = other RNA
taactagtggtcacagaatc

SEQ ID NO: 1910 - RNA, 20 nt, synthetic construct
  source 1..20: mol_type = other RNA
agttctgatacagtaactag

SEQ ID NO: 1911 - RNA, 20 nt, synthetic construct
  source 1..20: mol_type = other RNA
ttactgtatcagaactcatc

SEQ ID NO: 1912 - RNA, 20 nt, synthetic construct
  source 1..20: mol_type = other RNA
acttataaatagcactgatc

SEQ ID NO: 1913 - RNA, 20 nt, synthetic construct
  source 1..20: mol_type = other RNA
gatcagtgctatttataagt

SEQ ID NO: 1914 - RNA, 20 nt, synthetic construct
  source 1..20: mol_type = other RNA
agatcagtgctatttataag

SEQ ID NO: 1915 - RNA, 20 nt, synthetic construct
  source 1..20: mol_type = other RNA
ccatcactaacctgttttct

SEQ ID NO: 1916 - RNA, 20 nt, synthetic construct
  source 1..20: mol_type = other RNA
cctagaaaacaggttagtga

SEQ ID NO: 1917 - RNA, 20 nt, synthetic construct
  source 1..20: mol_type = other RNA
tacgctgggtcctagaaaac

SEQ ID NO: 1918 - RNA, 20 nt, synthetic construct
  source 1..20: mol_type = other RNA
atacaaatgctacatacgct

SEQ ID NO: 1919 - RNA, 20 nt, synthetic construct
  source 1..20: mol_type = other RNA
aatacaaatgctacatacgc

SEQ ID NO: 1920 - RNA, 20 nt, synthetic construct
  source 1..20: mol_type = other RNA
catttgtattgcagtttccc

SEQ ID NO: 1921 - RNA, 20 nt, synthetic construct
  source 1..20: mol_type = other RNA
tgcaaaacacaagtaagcca

SEQ ID NO: 1922 - RNA, 20 nt, synthetic construct
  source 1..20: mol_type = other RNA
gtgcaaaacacaagtaagcc

SEQ ID NO: 1923 - RNA, 20 nt, synthetic construct
  source 1..20: mol_type = other RNA
ttgcactgatgaattttgac

SEQ ID NO: 1924 - RNA, 20 nt, synthetic construct
  source 1..20: mol_type = other RNA
tgcactgatgaattttgaca

SEQ ID NO: 1925 - RNA, 20 nt, synthetic construct
  source 1..20: mol_type = other RNA
gcagtattgcacaagtaaag

SEQ ID NO: 1926 - RNA, 20 nt, synthetic construct
  source 1..20: mol_type = other RNA
aaaaagtataaaaatacagt

SEQ ID NO: 1927 - RNA, 20 nt, synthetic construct
  source 1..20: mol_type = other RNA
tactgtatttttatactttt

SEQ ID NO: 1928 - RNA, 20 nt, synthetic construct
  source 1..20: mol_type = other RNA
gtataaaaatacagtaggaa

SEQ ID NO: 1929 - RNA, 20 nt, synthetic construct
  source 1..20: mol_type = other RNA
atgtacaagaaataaattag

SEQ ID NO: 1930 - RNA, 20 nt, synthetic construct
  source 1..20: mol_type = other RNA
gatgtacaagaaataaatta

SEQ ID NO: 1931 - RNA, 20 nt, synthetic construct
  source 1..20: mol_type = other RNA
agatgtacaagaaataaatt

SEQ ID NO: 1932 - RNA, 20 nt, synthetic construct
  source 1..20: mol_type = other RNA
cacttaacacatccaattaa

SEQ ID NO: 1933 - RNA, 20 nt, synthetic construct
  source 1..20: mol_type = other RNA
gactttgcagaacctttaat

SEQ ID NO: 1934 - RNA, 20 nt, synthetic construct
  source 1..20: mol_type = other RNA
ggttctgcaaagtcttctgc

SEQ ID NO: 1935 - RNA, 20 nt, synthetic construct
  source 1..20: mol_type = other RNA
tctgcaaagtcttctgctgg

SEQ ID NO: 1936 - RNA, 20 nt, synthetic construct
  source 1..20: mol_type = other RNA
ctgcaaagtcttctgctggt

SEQ ID NO: 1937 - RNA, 20 nt, synthetic construct
  source 1..20: mol_type = other RNA
ggtgggtgctcttcatcccc

SEQ ID NO: 1938 - RNA, 20 nt, synthetic construct
  source 1..20: mol_type = other RNA
aaagtaaactttacatccag

SEQ ID NO: 1939 - RNA, 20 nt, synthetic construct
  source 1..20: mol_type = other RNA
caaagtaaactttacatcca

SEQ ID NO: 1940 - RNA, 20 nt, synthetic construct
  source 1..20: mol_type = other RNA
acaaagtaaactttacatcc

SEQ ID NO: 1941 - RNA, 20 nt, synthetic construct
  source 1..20: mol_type = other RNA
tttgtaaacaaacaactgtg

SEQ ID NO: 1942 - RNA, 20 nt, synthetic construct
  source 1..20: mol_type = other RNA
acaactgtgaggcaatctag

SEQ ID NO: 1943 - RNA, 20 nt, synthetic construct
  source 1..20: mol_type = other RNA
caactgtgaggcaatctaga

SEQ ID NO: 1944 - RNA, 20 nt, synthetic construct
  source 1..20: mol_type = other RNA
gcgagcctcactttagtttc

SEQ ID NO: 1945 - RNA, 20 nt, synthetic construct
  source 1..20: mol_type = other RNA
cctcactttagtttccggag

SEQ ID NO: 1946 - RNA, 20 nt, synthetic construct
  source 1..20: mol_type = other RNA
ctcactttagtttccggagt

SEQ ID NO: 1947 - RNA, 20 nt, synthetic construct
  source 1..20: mol_type = other RNA
ccactccggaaactaaagtg

SEQ ID NO: 1948 - RNA, 20 nt, synthetic construct
  source 1..20: mol_type = other RNA
tagtttccggagtgggcttc

SEQ ID NO: 1949 - RNA, 20 nt, synthetic construct
  source 1..20: mol_type = other RNA
gcaagacctgaagcccactc

SEQ ID NO: 1950 - RNA, 20 nt, synthetic construct
  source 1..20: mol_type = other RNA
ggtcttgctttgcacatcaa

SEQ ID NO: 1951 - RNA, 20 nt, synthetic construct
  source 1..20: mol_type = other RNA
attctcaagtcatgaatatt

SEQ ID NO: 1952 - RNA, 20 nt, synthetic construct
  source 1..20: mol_type = other RNA
tattaggtgtctgtcaatct

SEQ ID NO: 1953 - RNA, 20 nt, synthetic construct
  source 1..20: mol_type = other RNA
gacttcttattttatgtttt

SEQ ID NO: 1954 - RNA, 20 nt, synthetic construct
  source 1..20: mol_type = other RNA
tctatgttcgtctgtgtgtt

SEQ ID NO: 1955 - RNA, 20 nt, synthetic construct
  source 1..20: mol_type = other RNA
tagatgcacacaaacataaa

SEQ ID NO: 1956 - RNA, 20 nt, synthetic construct
  source 1..20: mol_type = other RNA
ggactaacaatgaactgaaa

SEQ ID NO: 1957 - RNA, 20 nt, synthetic construct
  source 1..20: mol_type = other RNA
gtatgaaagcaggatgtagg

SEQ ID NO: 1958 - RNA, 20 nt, synthetic construct
  source 1..20: mol_type = other RNA
aaagtatgaaagcaggatgt

SEQ ID NO: 1959 - RNA, 20 nt, synthetic construct
  source 1..20: mol_type = other RNA
tatgttgaaagtatgaaagc

SEQ ID NO: 1960 - RNA, 20 nt, synthetic construct
  source 1..20: mol_type = other RNA
aacataatttaacacattca

SEQ ID NO: 1961 - RNA, 20 nt, synthetic construct
  source 1..20: mol_type = other RNA
aaaatatctatctataccaa

SEQ ID NO: 1962 - RNA, 20 nt, synthetic construct
  source 1..20: mol_type = other RNA
aaaaaaagtttgaaaaccat

SEQ ID NO: 1963 - RNA, 20 nt, synthetic construct
  source 1..20: mol_type = other RNA
cgaagtcttgctctgttgcc

SEQ ID NO: 1964 - RNA, 20 nt, synthetic construct
  source 1..20: mol_type = other RNA
gtcttgctctgttgccaggc

SEQ ID NO: 1965 - RNA, 20 nt, synthetic construct
  source 1..20: mol_type = other RNA
gttgccaggctggagtgcag

SEQ ID NO: 1966 - RNA, 20 nt, synthetic construct
  source 1..20: mol_type = other RNA
tgcaccactgcactccagcc

SEQ ID NO: 1967 - RNA, 20 nt, synthetic construct
  source 1..20: mol_type = other RNA
ggagtgcagtggtgcaatct

SEQ ID NO: 1968 - RNA, 20 nt, synthetic construct
  source 1..20: mol_type = other RNA
tcactgcaacctctgcctcc

SEQ ID NO: 1969 - RNA, 20 nt, synthetic construct
  source 1..20: mol_type = other RNA
cactgcaacctctgcctccc

SEQ ID NO: 1970 - RNA, 20 nt, synthetic construct
  source 1..20: mol_type = other RNA
cacttgaacccgggaggcag

SEQ ID NO: 1971 - RNA, 20 nt, synthetic construct
  source 1..20: mol_type = other RNA
gagaatcacttgaacccggg

SEQ ID NO: 1972 - RNA, 20 nt, synthetic construct
  source 1..20: mol_type = other RNA
caggagaatcacttgaaccc

SEQ ID NO: 1973 - RNA, 20 nt, synthetic construct
  source 1..20: mol_type = other RNA
gcaggagaatcacttgaacc

SEQ ID NO: 1974 - RNA, 20 nt, synthetic construct
  source 1..20: mol_type = other RNA
tctcctgccttagcctccca

SEQ ID NO: 1975 - RNA, 20 nt, synthetic construct
  source 1..20: mol_type = other RNA
gccttagcctcccaaggagc

SEQ ID NO: 1976 - RNA, 20 nt, synthetic construct
  source 1..20: mol_type = other RNA
ccttagcctcccaaggagct

SEQ ID NO: 1977 - RNA, 20 nt, synthetic construct
  source 1..20: mol_type = other RNA
gctccttgggaggctaaggc

SEQ ID NO: 1978 - RNA, 20 nt, synthetic construct
  source 1..20: mol_type = other RNA
cccagctccttgggaggcta

SEQ ID NO: 1979 - RNA, 20 nt, synthetic construct
  source 1..20: mol_type = other RNA
tcccaaggagctgggactac

SEQ ID NO: 1980 - RNA, 20 nt, synthetic construct
  source 1..20: mol_type = other RNA
tgtagtcccagctccttggg

SEQ ID NO: 1981 - RNA, 20 nt, synthetic construct
  source 1..20: mol_type = other RNA
gcctgtagtcccagctcctt

SEQ ID NO: 1982 - RNA, 20 nt, synthetic construct
  source 1..20: mol_type = other RNA
tgcctgtagtcccagctcct

SEQ ID NO: 1983 - RNA, 20 nt, synthetic construct
  source 1..20: mol_type = other RNA
caaaaattatctgggcgtgg

SEQ ID NO: 1984 - RNA, 20 nt, synthetic construct
  source 1..20: mol_type = other RNA
atacaaaaattatctgggcg

SEQ ID NO: 1985 - RNA, 20 nt, synthetic construct
  source 1..20: mol_type = other RNA
taaaaatacaaaaattatct

SEQ ID NO: 1986 - RNA, 20 nt, synthetic construct
  source 1..20: mol_type = other RNA
ctaaaaatacaaaaattatc

SEQ ID NO: 1987 - RNA, 20 nt, synthetic construct
  source 1..20: mol_type = other RNA
ttttgtatttttagtaaaga

SEQ ID NO: 1988 - RNA, 20 nt, synthetic construct
  source 1..20: mol_type = other RNA
tttgtatttttagtaaagaa

SEQ ID NO: 1989 - RNA, 20 nt, synthetic construct
  source 1..20: mol_type = other RNA
aagaagggatttcaccatgt

SEQ ID NO: 1990 - RNA, 20 nt, synthetic construct
  source 1..20: mol_type = other RNA
gggatttcaccatgttggcc

SEQ ID NO: 1991 - RNA, 20 nt, synthetic construct
  source 1..20: mol_type = other RNA
ggagactgtcctggccaaca

SEQ ID NO: 1992 - RNA, 20 nt, synthetic construct
  source 1..20: mol_type = other RNA
tcaagagatggagactgtcc

SEQ ID NO: 1993 - RNA, 20 nt, synthetic construct
  source 1..20: mol_type = other RNA
cggatcacgaggtcaagaga

SEQ ID NO: 1994 - RNA, 20 nt, synthetic construct
  source 1..20: mol_type = other RNA
acctcgtgatccgcccgcct

SEQ ID NO: 1995 - RNA, 20 nt, synthetic construct
  source 1..20: mol_type = other RNA
gccaaggcgggcggatcacg

SEQ ID NO: 1996 - RNA, 20 nt, synthetic construct
  source 1..20: mol_type = other RNA
cttcggaaggccaaggcggg

SEQ ID NO: 1997 - RNA, 20 nt, synthetic construct
  source 1..20: mol_type = other RNA
gccttggccttccgaagtgc

SEQ ID NO: 1998 - RNA, 20 nt, synthetic construct
  source 1..20: mol_type = other RNA
ccttggccttccgaagtgct

SEQ ID NO: 1999 - RNA, 20 nt, synthetic construct
  source 1..20: mol_type = other RNA
gcacttcggaaggccaaggc

SEQ ID NO: 2000 - RNA, 20 nt, synthetic construct
  source 1..20: mol_type = other RNA
agcacttcggaaggccaagg

SEQ ID NO: 2001 - RNA, 20 nt, synthetic construct
  source 1..20: mol_type = other RNA
cccagcacttcggaaggcca

SEQ ID NO: 2002 - RNA, 20 nt, synthetic construct
  source 1..20: mol_type = other RNA
tgtaatcccagcacttcgga

SEQ ID NO: 2003 - RNA, 20 nt, synthetic construct
  source 1..20: mol_type = other RNA
cgcttgtaatcccagcactt

SEQ ID NO: 2004 - RNA, 20 nt, synthetic construct
  source 1..20: mol_type = other RNA
caagcgtgagccaccacacc

SEQ ID NO: 2005 - RNA, 20 nt, synthetic construct
  source 1..20: mol_type = other RNA
acagtttgggccgggtgtgg

SEQ ID NO: 2006 - RNA, 20 nt, synthetic construct
  source 1..20: mol_type = other RNA
aaaacagtttgggccgggtg

SEQ ID NO: 2007 - RNA, 20 nt, synthetic construct
  source 1..20: mol_type = other RNA
caaaaaaaacagtttgggcc

SEQ ID NO: 2008 - RNA, 20 nt, synthetic construct
  source 1..20: mol_type = other RNA
acaaaaaaaacagtttgggc

SEQ ID NO: 2009 - RNA, 20 nt, synthetic construct
  source 1..20: mol_type = other RNA
acaaacaaaaaaaacagttt

SEQ ID NO: 2010 - RNA, 20 nt, synthetic construct
  source 1..20: mol_type = other RNA
aacaaacaaaaaaaacagtt

SEQ ID NO: 2011 - RNA, 20 nt, synthetic construct
  source 1..20: mol_type = other RNA
tttgtttgtttcttttgaga

SEQ ID NO: 2012 - RNA, 20 nt, synthetic construct
  source 1..20: mol_type = other RNA
ggagtctcgctctgtcgccc

SEQ ID NO: 2013 - RNA, 20 nt, synthetic construct
  source 1..20: mol_type = other RNA
tctcgctctgtcgccctggc

SEQ ID NO: 2014 - RNA, 20 nt, synthetic construct
  source 1..20: mol_type = other RNA
acgtcactgcactccagcca

SEQ ID NO: 2015 - RNA, 20 nt, synthetic construct
  source 1..20: mol_type = other RNA
cacgtcactgcactccagcc

SEQ ID NO: 2016 - RNA, 20 nt, synthetic construct
  source 1..20: mol_type = other RNA
tcactgcaacctccatctcc

SEQ ID NO: 2017 - RNA, 20 nt, synthetic construct
  source 1..20: mol_type = other RNA
cactgcaacctccatctcct

SEQ ID NO: 2018 - RNA, 20 nt, synthetic construct
  source 1..20: mol_type = other RNA
tgcttgaacccaggagatgg

SEQ ID NO: 2019 - RNA, 20 nt, synthetic construct
  source 1..20: mol_type = other RNA
aattgcttgaacccaggaga

SEQ ID NO: 2020 - RNA, 20 nt, synthetic construct
  source 1..20: mol_type = other RNA
taggagaattgcttgaaccc

SEQ ID NO: 2021 - RNA, 20 nt, synthetic construct
  source 1..20: mol_type = other RNA
gctactcaggaggctgaggt

SEQ ID NO: 2022 - RNA, 20 nt, synthetic construct
  source 1..20: mol_type = other RNA
ctcagctactcaggaggctg

SEQ ID NO: 2023 - RNA, 20 nt, synthetic construct
  source 1..20: mol_type = other RNA
tcctgagtagctgagattac

SEQ ID NO: 2024 - RNA, 20 nt, synthetic construct
  source 1..20: mol_type = other RNA
tgtaatctcagctactcagg

SEQ ID NO: 2025 - RNA, 20 nt, synthetic construct
  source 1..20: mol_type = other RNA
acctgtaatctcagctactc

SEQ ID NO: 2026 - RNA, 20 nt, synthetic construct
  source 1..20: mol_type = other RNA
aattagctgggcatggtgga

SEQ ID NO: 2027 - RNA, 20 nt, synthetic construct
  source 1..20: mol_type = other RNA
aaattagctgggcatggtgg

SEQ ID NO: 2028 - RNA, 20 nt, synthetic construct
  source 1..20: mol_type = other RNA
caaaaattagctgggcatgg

SEQ ID NO: 2029 - RNA, 20 nt, synthetic construct
  source 1..20: mol_type = other RNA
atgcaaaaattagctgggca

SEQ ID NO: 2030 - RNA, 20 nt, synthetic construct
  source 1..20: mol_type = other RNA
taaaaatgcaaaaattagct

SEQ ID NO: 2031 - RNA, 20 nt, synthetic construct
  source 1..20: mol_type = other RNA
ctaaaaatgcaaaaattagc

SEQ ID NO: 2032 - RNA, 20 nt, synthetic construct
  source 1..20: mol_type = other RNA
ttttgcatttttagtagaga

SEQ ID NO: 2033 - RNA, 20 nt, synthetic construct
  source 1..20: mol_type = other RNA
gagatggtgtttcaccacgt

SEQ ID NO: 2034 - RNA, 20 nt, synthetic construct
  source 1..20: mol_type = other RNA
ggtgtttcaccacgttggcc

SEQ ID NO: 2035 - RNA, 20 nt, synthetic construct
  source 1..20: mol_type = other RNA
tttcaccacgttggccaggc

SEQ ID NO: 2036 - RNA, 20 nt, synthetic construct
  source 1..20: mol_type = other RNA
caagaccagcctggccaacg

SEQ ID NO: 2037 - RNA, 20 nt, synthetic construct
  source 1..20: mol_type = other RNA
tcaggagttcaagaccagcc

SEQ ID NO: 2038 - RNA, 20 nt, synthetic construct
  source 1..20: mol_type = other RNA
ggtcttgaactcctgacctc

SEQ ID NO: 2039 - RNA, 20 nt, synthetic construct
  source 1..20: mol_type = other RNA
tgggcagatcacctgaggtc

SEQ ID NO: 2040 - RNA, 20 nt, synthetic construct
  source 1..20: mol_type = other RNA
tgaagtgggcagatcacctg

SEQ ID NO: 2041 - RNA, 20 nt, synthetic construct
  source 1..20: mol_type = other RNA
acttcagcctcccaaagtgc

SEQ ID NO: 2042 - RNA, 20 nt, synthetic construct
  source 1..20: mol_type = other RNA
cttcagcctcccaaagtgct

SEQ ID NO: 2043 - RNA, 20 nt, synthetic construct
  source 1..20: mol_type = other RNA
gcactttgggaggctgaagt

SEQ ID NO: 2044 - RNA, 20 nt, synthetic construct
  source 1..20: mol_type = other RNA
agcactttgggaggctgaag

SEQ ID NO: 2045 - RNA, 20 nt, synthetic construct
  source 1..20: mol_type = other RNA
tcccaaagtgctgggattac

SEQ ID NO: 2046 - RNA, 20 nt, synthetic construct
  source 1..20: mol_type = other RNA
tgtaatcccagcactttggg

SEQ ID NO: 2047 - RNA, 20 nt, synthetic construct
  source 1..20: mol_type = other RNA
gcctgtaatcccagcacttt

SEQ ID NO: 2048 - RNA, 20 nt, synthetic construct
  source 1..20: mol_type = other RNA
tgcctgtaatcccagcactt

SEQ ID NO: 2049 - RNA, 20 nt, synthetic construct
  source 1..20: mol_type = other RNA
aacagtttggtcgggcgcgg

SEQ ID NO: 2050 - RNA, 20 nt, synthetic construct
  source 1..20: mol_type = other RNA
aaaaacagtttggtcgggcg

SEQ ID NO: 2051 - RNA, 20 nt, synthetic construct
  source 1..20: mol_type = other RNA
catttaaaaacagtttggtc

SEQ ID NO: 2052 - RNA, 20 nt, synthetic construct
  source 1..20: mol_type = other RNA
tcatttaaaaacagtttggt

SEQ ID NO: 2053 - RNA, 20 nt, synthetic construct
  source 1..20: mol_type = other RNA
gttatcatttaaaaacagtt

SEQ ID NO: 2054 - RNA, 20 nt, synthetic construct
  source 1..20: mol_type = other RNA
aggcttaagtattttaaagg

SEQ ID NO: 2055 - RNA, 20 nt, synthetic construct
  source 1..20: mol_type = other RNA
aaggcttaagtattttaaag

SEQ ID NO: 2056 - RNA, 20 nt, synthetic construct
  source 1..20: mol_type = other RNA
taaggcttaagtattttaaa

SEQ ID NO: 2057 - RNA, 20 nt, synthetic construct
  source 1..20: mol_type = other RNA
ataaggcttaagtattttaa

SEQ ID NO: 2058 - RNA, 20 nt, synthetic construct
  source 1..20: mol_type = other RNA
ccttatgcagaaatcttatg

SEQ ID NO: 2059 - RNA, 20 nt, synthetic construct
  source 1..20: mol_type = other RNA
ccacataagatttctgcata

SEQ ID NO: 2060 - RNA, 20 nt, synthetic construct
  source 1..20: mol_type = other RNA
atgtggcatataaagagaca

SEQ ID NO: 2061 - RNA, 20 nt, synthetic construct
  source 1..20: mol_type = other RNA
gagacaaggcagagatgctg

SEQ ID NO: 2062 - RNA, 20 nt, synthetic construct
  source 1..20: mol_type = other RNA
aagtaacctcttgacccacc

SEQ ID NO: 2063 - RNA, 20 nt, synthetic construct
  source 1..20: mol_type = other RNA
ggatgtccaggtgggtcaag

SEQ ID NO: 2064 - RNA, 20 nt, synthetic construct
  source 1..20: mol_type = other RNA
tgctcattggatgtccaggt

SEQ ID NO: 2065 - RNA, 20 nt, synthetic construct
  source 1..20: mol_type = other RNA
atgctcattggatgtccagg

SEQ ID NO: 2066 - RNA, 20 nt, synthetic construct
  source 1..20: mol_type = other RNA
actatgctcattggatgtcc

SEQ ID NO: 2067 - RNA, 20 nt, synthetic construct
  source 1..20: mol_type = other RNA
ggttttcaaactatgctcat

SEQ ID NO: 2068 - RNA, 20 nt, synthetic construct
  source 1..20: mol_type = other RNA
gtttgaaaaccactgaaata

SEQ ID NO: 2069 - RNA, 20 nt, synthetic construct
  source 1..20: mol_type = other RNA
gatagcataccttatttcag

SEQ ID NO: 2070 - RNA, 20 nt, synthetic construct
  source 1..20: mol_type = other RNA
atggatagcatacattatta

SEQ ID NO: 2071 - RNA, 20 nt, synthetic construct
  source 1..20: mol_type = other RNA
aatttaattgctaggaggca

SEQ ID NO: 2072 - RNA, 20 nt, synthetic construct
  source 1..20: mol_type = other RNA
ttacaaatttaattgctagg

SEQ ID NO: 2073 - RNA, 20 nt, synthetic construct
  source 1..20: mol_type = other RNA
ttgttacaaatttaattgct

SEQ ID NO: 2074 - RNA, 20 nt, synthetic construct
  source 1..20: mol_type = other RNA
aagacaaattaaacactgaa

SEQ ID NO: 2075 - RNA, 20 nt, synthetic construct
  source 1..20: mol_type = other RNA
gaatggaatgttgaaatctg

SEQ ID NO: 2076 - RNA, 20 nt, synthetic construct
  source 1..20: mol_type = other RNA
taagttaaaatgacaatgta

SEQ ID NO: 2077 - RNA, 20 nt, synthetic construct
  source 1..20: mol_type = other RNA
gttggggtagattatgattt

SEQ ID NO: 2078 - RNA, 20 nt, synthetic construct
  source 1..20: mol_type = other RNA
tgaaaatttcaatgtagttg

SEQ ID NO: 2079 - RNA, 20 nt, synthetic construct
  source 1..20: mol_type = other RNA
atgaaaatttcaatgtagtt

SEQ ID NO: 2080 - RNA, 20 nt, synthetic construct
  source 1..20: mol_type = other RNA
catgaaaatttcaatgtagt

SEQ ID NO: 2081 - RNA, 20 nt, synthetic construct
  source 1..20: mol_type = other RNA
aaaaataaacatatcaataa

SEQ ID NO: 2082 - RNA, 20 nt, synthetic construct
  source 1..20: mol_type = other RNA
aaaataaacatatcaataat

SEQ ID NO: 2083 - RNA, 20 nt, synthetic construct
  source 1..20: mol_type = other RNA
tcaagactttgtaaagaaat

SEQ ID NO: 2084 - RNA, 20 nt, synthetic construct
  source 1..20: mol_type = other RNA
gggatagtcaggtaaacagt

SEQ ID NO: 2085 - RNA, 20 nt, synthetic construct
  source 1..20: mol_type = other RNA
tttacctgactatcccagta

SEQ ID NO: 2086 - RNA, 20 nt, synthetic construct
  source 1..20: mol_type = other RNA
ttctccttactgggatagtc

SEQ ID NO: 2087 - RNA, 20 nt, synthetic construct
  source 1..20: mol_type = other RNA
gaaggaaaattctccttact

SEQ ID NO: 2088 - RNA, 20 nt, synthetic construct
  source 1..20: mol_type = other RNA
tgaaggaaaattctccttac

SEQ ID NO: 2089 - RNA, 20 nt, synthetic construct
  source 1..20: mol_type = other RNA
tttccttcaaagatattttt

SEQ ID NO: 2090 - RNA, 20 nt, synthetic construct
  source 1..20: mol_type = other RNA
tttcctaaaaatatctttga

SEQ ID NO: 2091 - RNA, 20 nt, synthetic construct
  source 1..20: mol_type = other RNA
gtttgcttttctttttaaaa

SEQ ID NO: 2092 - RNA, 20 nt, synthetic construct
  source 1..20: mol_type = other RNA
tttgcttttctttttaaaat

SEQ ID NO: 2093 - RNA, 20 nt, synthetic construct
  source 1..20: mol_type = other RNA
ttgcttttctttttaaaatg

SEQ ID NO: 2094 - RNA, 20 nt, synthetic construct
  source 1..20: mol_type = other RNA
tgatatgagcagttagaagt

SEQ ID NO: 2095 - RNA, 20 nt, synthetic construct
  source 1..20: mol_type = other RNA
caaacttctctttagaaaaa

SEQ ID NO: 2096 - RNA, 20 nt, synthetic construct
  source 1..20: mol_type = other RNA
gtatgtcgattgaattgtac

SEQ ID NO: 2097 - RNA, 20 nt, synthetic construct
  source 1..20: mol_type = other RNA
ttttattcttaagcatttca

SEQ ID NO: 2098 - RNA, 20 nt, synthetic construct
  source 1..20: mol_type = other RNA
cttttattcttaagcatttc

SEQ ID NO: 2099 - RNA, 20 nt, synthetic construct
  source 1..20: mol_type = other RNA
gtataatgtactattgacat

SEQ ID NO: 2100 - RNA, 20 nt, synthetic construct
  source 1..20: mol_type = other RNA
tgtataatgtactattgaca

SEQ ID NO: 2101 - RNA, 20 nt, synthetic construct
  source 1..20: mol_type = other RNA
tgtggttttatctacgttat

SEQ ID NO: 2102 - RNA, 20 nt, synthetic construct
  source 1..20: mol_type = other RNA
gatataagcaataaatattg

SEQ ID NO: 2103 - RNA, 20 nt, synthetic construct
  source 1..20: mol_type = other RNA
ttattgcttatatcaagtgc

SEQ ID NO: 2104 - RNA, 20 nt, synthetic construct
  source 1..20: mol_type = other RNA
atttgtttttggaggctatc

SEQ ID NO: 2105 - RNA, 20 nt, synthetic construct
  source 1..20: mol_type = other RNA
atcacaggatttgtttttgg

SEQ ID NO: 2106 - RNA, 20 nt, synthetic construct
  source 1..20: mol_type = other RNA
tttatcacaggatttgtttt

SEQ ID NO: 2107 - RNA, 20 nt, synthetic construct
  source 1..20: mol_type = other RNA
attgagatatcctttatcac

SEQ ID NO: 2108 - RNA, 20 nt, synthetic construct
  source 1..20: mol_type = other RNA
aggatatctcaatgttggtc

SEQ ID NO: 2109 - RNA, 20 nt, synthetic construct
  source 1..20: mol_type = other RNA
cattcatgtttgttaaaaac

SEQ ID NO: 2110 - RNA, 20 nt, synthetic construct
  source 1..20: mol_type = other RNA
ttagacagccatttacagtt

SEQ ID NO: 2111 - RNA, 20 nt, synthetic construct
  source 1..20: mol_type = other RNA
tagacagccatttacagttt

SEQ ID NO: 2112 - RNA, 20 nt, synthetic construct
  source 1..20: mol_type = other RNA
agacagccatttacagtttg

SEQ ID NO: 2113 - RNA, 20 nt, synthetic construct
  source 1..20: mol_type = other RNA
atttacagtttggggttcag

SEQ ID NO: 2114 - RNA, 20 nt, synthetic construct
  source 1..20: mol_type = other RNA
tctgaaccccaaactgtaaa

SEQ ID NO: 2115 - RNA, 20 nt, synthetic construct
  source 1..20: mol_type = other RNA
agtcaagagtcctgagatgt

SEQ ID NO: 2116 - RNA, 20 nt, synthetic construct
  source 1..20: mol_type = other RNA
gtcaagagtcctgagatgtt

SEQ ID NO: 2117 - RNA, 20 nt, synthetic construct
  source 1..20: mol_type = other RNA
agtcacaagcccaacatctc

SEQ ID NO: 2118 - RNA, 20 nt, synthetic construct
  source 1..20: mol_type = other RNA
gactgtaaatatcacttatc

SEQ ID NO: 2119 - RNA, 20 nt, synthetic construct
  source 1..20: mol_type = other RNA
ctattctactgcaccgtttt

SEQ ID NO: 2120 - RNA, 20 nt, synthetic construct
  source 1..20: mol_type = other RNA
tattctactgcaccgttttt

SEQ ID NO: 2121 - RNA, 20 nt, synthetic construct
  source 1..20: mol_type = other RNA
tgcaccgtttttgggatatg

SEQ ID NO: 2122 - RNA, 20 nt, synthetic construct
  source 1..20: mol_type = other RNA
aacgcctcatatcccaaaaa

SEQ ID NO: 2123 - RNA, 20 nt, synthetic construct
  source 1..20: mol_type = other RNA
cagtgctacattaatcatag

SEQ ID NO: 2124 - RNA, 20 nt, synthetic construct
  source 1..20: mol_type = other RNA
acagtgctacattaatcata

SEQ ID NO: 2125 - RNA, 20 nt, synthetic construct
  source 1..20: mol_type = other RNA
gacagtgctacattaatcat

SEQ ID NO: 2126 - RNA, 20 nt, synthetic construct
  source 1..20: mol_type = other RNA
ttactagtgcagaagcttgc

SEQ ID NO: 2127 - RNA, 20 nt, synthetic construct
  source 1..20: mol_type = other RNA
tactagtgcagaagcttgct

SEQ ID NO: 2128 - RNA, 20 nt, synthetic construct
  source 1..20: mol_type = other RNA
gggcaaaattaattgtttat

SEQ ID NO: 2129 - RNA, 20 nt, synthetic construct
  source 1..20: mol_type = other RNA
ggcaaaattaattgtttata

SEQ ID NO: 2130 - RNA, 20 nt, synthetic construct
  source 1..20: mol_type = other RNA
tggttggcgcttttgttggc

SEQ ID NO: 2131 - RNA, 20 nt, synthetic construct
  source 1..20: mol_type = other RNA
attttggttggcgcttttgt

SEQ ID NO: 2132 - RNA, 20 nt, synthetic construct
  source 1..20: mol_type = other RNA
tttatgtcagtcattttggt

SEQ ID NO: 2133 - RNA, 20 nt, synthetic construct
  source 1..20: mol_type = other RNA
ggggtttatgtcagtcattt

SEQ ID NO: 2134 - RNA, 20 nt, synthetic construct
  source 1..20: mol_type = other RNA
aaccccatcttagtgagaat

SEQ ID NO: 2135 - RNA, 20 nt, synthetic construct
  source 1..20: mol_type = other RNA
aacctattctcactaagatg

SEQ ID NO: 2136 - RNA, 20 nt, synthetic construct
  source 1..20: mol_type = other RNA
caacctattctcactaagat

SEQ ID NO: 2137 - RNA, 20 nt, synthetic construct
  source 1..20: mol_type = other RNA
gcaacctattctcactaaga

SEQ ID NO: 2138 - RNA, 20 nt, synthetic construct
  source 1..20: mol_type = other RNA
aaagaaaaaggtggttatat

SEQ ID NO: 2139 - RNA, 20 nt, synthetic construct
  source 1..20: mol_type = other RNA
atgaacgaaaaagaaaaagg

SEQ ID NO: 2140 - RNA, 20 nt, synthetic construct
  source 1..20: mol_type = other RNA
agaatgaacgaaaaagaaaa

SEQ ID NO: 2141 - RNA, 20 nt, synthetic construct
  source 1..20: mol_type = other RNA
aaaggaagtgcacacagagc

SEQ ID NO: 2142 - RNA, 20 nt, synthetic construct
  source 1..20: mol_type = other RNA
acttgagtactctaacacag

SEQ ID NO: 2143 - RNA, 20 nt, synthetic construct
  source 1..20: mol_type = other RNA
tactctaacacagaggacct

SEQ ID NO: 2144 - RNA, 20 nt, synthetic construct
  source 1..20: mol_type = other RNA
ggatggttttatttgcgcct

SEQ ID NO: 2145 - RNA, 20 nt, synthetic construct
  source 1..20: mol_type = other RNA
tagggtgaaaactatgtgga

SEQ ID NO: 2146 - RNA, 20 nt, synthetic construct
  source 1..20: mol_type = other RNA
caaatagggtgaaaactatg

SEQ ID NO: 2147 - RNA, 20 nt, synthetic construct
  source 1..20: mol_type = other RNA
ttttcaccctatttgaacac

SEQ ID NO: 2148 - RNA, 20 nt, synthetic construct
  source 1..20: mol_type = other RNA
aggtatgtaatttttatatt

SEQ ID NO: 2149 - RNA, 20 nt, synthetic construct
  source 1..20: mol_type = other RNA
attacatacctgaaatccta

SEQ ID NO: 2150 - RNA, 20 nt, synthetic construct
  source 1..20: mol_type = other RNA
acctgaaatcctatggcacc

SEQ ID NO: 2151 - RNA, 20 nt, synthetic construct
  source 1..20: mol_type = other RNA
accaggtgccataggatttc

SEQ ID NO: 2152 - RNA, 20 nt, synthetic construct
  source 1..20: mol_type = other RNA
tttatgggaccaggtgccat

SEQ ID NO: 2153 - RNA, 20 nt, synthetic construct
  source 1..20: mol_type = other RNA
aaaataaattttatgggacc

SEQ ID NO: 2154 - RNA, 20 nt, synthetic construct
  source 1..20: mol_type = other RNA
attttaaaaataaattttat

SEQ ID NO: 2155 - RNA, 20 nt, synthetic construct
  source 1..20: mol_type = other RNA
tattttaaaaataaatttta

SEQ ID NO: 2156 - RNA, 20 nt, synthetic construct
  source 1..20: mol_type = other RNA
taactacaggctgaaagatg

SEQ ID NO: 2157 - RNA, 20 nt, synthetic construct
  source 1..20: mol_type = other RNA
ttcataaatttttttattta

SEQ ID NO: 2158 - RNA, 20 nt, synthetic construct
  source 1..20: mol_type = other RNA
ggttttcttaacttgaatat

SEQ ID NO: 2159 - RNA, 20 nt, synthetic construct
  source 1..20: mol_type = other RNA
agagtgtatttgaatttttg

SEQ ID NO: 2160 - RNA, 20 nt, synthetic construct
  source 1..20: mol_type = other RNA
cactctttgaaacaaagaca

SEQ ID NO: 2161 - RNA, 20 nt, synthetic construct
  source 1..20: mol_type = other RNA
actctttgaaacaaagacaa

SEQ ID NO: 2162 - RNA, 20 nt, synthetic construct
  source 1..20: mol_type = other RNA
aacaaagacaagggctcaag

SEQ ID NO: 2163 - RNA, 20 nt, synthetic construct
  source 1..20: mol_type = other RNA
aatgagacaagtcttgttat

SEQ ID NO: 2164 - RNA, 20 nt, synthetic construct
  source 1..20: mol_type = other RNA
aagtcttgttattggaaccc

SEQ ID NO: 2165 - RNA, 20 nt, synthetic construct
  source 1..20: mol_type = other RNA
ttgcattgattctgtttcct

SEQ ID NO: 2166 - RNA, 20 nt, synthetic construct
  source 1..20: mol_type = other RNA
cttgcattgattctgtttcc

SEQ ID NO: 2167 - RNA, 20 nt, synthetic construct
  source 1..20: mol_type = other RNA
aattatcgttgttctttcag

SEQ ID NO: 2168 - RNA, 20 nt, synthetic construct
  source 1..20: mol_type = other RNA
aagttgaaaaacctcagttc

SEQ ID NO: 2169 - RNA, 20 nt, synthetic construct
  source 1..20: mol_type = other RNA
agttgaaaaacctcagttct

SEQ ID NO: 2170 - RNA, 20 nt, synthetic construct
  source 1..20: mol_type = other RNA
gatgctgtatcccagaactg

SEQ ID NO: 2171 - RNA, 20 nt, synthetic construct
  source 1..20: mol_type = other RNA
cagagtttattcactgccag

SEQ ID NO: 2172 - RNA, 20 nt, synthetic construct
  source 1..20: mol_type = other RNA
tttttttaaattgcttccac

SEQ ID NO: 2173 - RNA, 20 nt, synthetic construct
  source 1..20: mol_type = other RNA
actctaaaaagtgaaaatca

SEQ ID NO: 2174 - RNA, 20 nt, synthetic construct
  source 1..20: mol_type = other RNA
ctctaaaaagtgaaaatcaa

SEQ ID NO: 2175 - RNA, 20 nt, synthetic construct
  source 1..20: mol_type = other RNA
ttgattttcactttttagag

SEQ ID NO: 2176 - RNA, 20 nt, synthetic construct
  source 1..20: mol_type = other RNA
ataattctttaaagccatat

SEQ ID NO: 2177 - RNA, 20 nt, synthetic construct
  source 1..20: mol_type = other RNA
catagtataaacagcctata

SEQ ID NO: 2178 - RNA, 20 nt, synthetic construct
  source 1..20: mol_type = other RNA
ttttttttttttttttgaga

SEQ ID NO: 2179 - RNA, 20 nt, synthetic construct
  source 1..20: mol_type = other RNA
tcttaatttctactgcaaaa

SEQ ID NO: 2180 - RNA, 20 nt, synthetic construct
  source 1..20: mol_type = other RNA
tgtcccagactcagtatata

SEQ ID NO: 2181 - RNA, 20 nt, synthetic construct
  source 1..20: mol_type = other RNA
ataccttatatactgagtct

SEQ ID NO: 2182 - RNA, 20 nt, synthetic construct
  source 1..20: mol_type = other RNA
tataccttatatactgagtc

SEQ ID NO: 2183 - RNA, 20 nt, synthetic construct
  source 1..20: mol_type = other RNA
attacaaattaaaatgatca

SEQ ID NO: 2184 - RNA, 20 nt, synthetic construct
  source 1..20: mol_type = other RNA
atgatcattttaatttgtaa

SEQ ID NO: 2185 - RNA, 20 nt, synthetic construct
  source 1..20: mol_type = other RNA
atttatttttaaattaatta

SEQ ID NO: 2186 - RNA, 20 nt, synthetic construct
  source 1..20: mol_type = other RNA
agtgaacaaagccagactaa

SEQ ID NO: 2187 - RNA, 20 nt, synthetic construct
  source 1..20: mol_type = other RNA
gtttgataagcacatgcatt

SEQ ID NO: 2188 - RNA, 20 nt, synthetic construct
  source 1..20: mol_type = other RNA
tcatataaagtccacaattt

SEQ ID NO: 2189 - RNA, 20 nt, synthetic construct
  source 1..20: mol_type = other RNA
catataaagtccacaatttc

SEQ ID NO: 2190 - RNA, 20 nt, synthetic construct
  source 1..20: mol_type = other RNA
aaattgtggactttatatga

SEQ ID NO: 2191 - RNA, 20 nt, synthetic construct
  source 1..20: mol_type = other RNA
tccacaatttcgggcaagaa

SEQ ID NO: 2192 - RNA, 20 nt, synthetic construct
  source 1..20: mol_type = other RNA
acctttcttgcccgaaattg

SEQ ID NO: 2193 - RNA, 20 nt, synthetic construct
  source 1..20: mol_type = other RNA
gttttcattttttaacttta

SEQ ID NO: 2194 - RNA, 20 nt, synthetic construct
  source 1..20: mol_type = other RNA
aaatatagcatgtatatatc

SEQ ID NO: 2195 - RNA, 20 nt, synthetic construct
  source 1..20: mol_type = other RNA
cgctagcctttagcaattaa

SEQ ID NO: 2196 - RNA, 20 nt, synthetic construct
  source 1..20: mol_type = other RNA
ctttaattgctaaaggctag

SEQ ID NO: 2197 - RNA, 20 nt, synthetic construct
  source 1..20: mol_type = other RNA
ttttggcctttaattgctaa

SEQ ID NO: 2198 - RNA, 20 nt, synthetic construct
  source 1..20: mol_type = other RNA
gcaattaaaggccaaaacta

SEQ ID NO: 2199 - RNA, 20 nt, synthetic construct
  source 1..20: mol_type = other RNA
caaaactaaggaatgaatat

SEQ ID NO: 2200 - RNA, 20 nt, synthetic construct
  source 1..20: mol_type = other RNA
caatattcattccttagttt

SEQ ID NO: 2201 - RNA, 20 nt, synthetic construct
  source 1..20: mol_type = other RNA
atataaagattttcattttg

SEQ ID NO: 2202 - RNA, 20 nt, synthetic construct
  source 1..20: mol_type = other RNA
catataaagattttcatttt

SEQ ID NO: 2203 - RNA, 20 nt, synthetic construct
  source 1..20: mol_type = other RNA
gcatataaagattttcattt

SEQ ID NO: 2204 - RNA, 20 nt, synthetic construct
  source 1..20: mol_type = other RNA
ctctctcctctctcttcaca

SEQ ID NO: 2205 - RNA, 20 nt, synthetic construct
  source 1..20: mol_type = other RNA
tctctctcctctctcttcac

SEQ ID NO: 2206 - RNA, 20 nt, synthetic construct
  source 1..20: mol_type = other RNA
gagaggagagagagcagatg

SEQ ID NO: 2207 - RNA, 20 nt, synthetic construct
  source 1..20: mol_type = other RNA
agaggagagagagcagatga

SEQ ID NO: 2208 - RNA, 20 nt, synthetic construct
  source 1..20: mol_type = other RNA
ggaagcagacagaaagagca

SEQ ID NO: 2209 - RNA, 20 nt, synthetic construct
  source 1..20: mol_type = other RNA
gacagaaagagcaaggctcc

SEQ ID NO: 2210 - RNA, 20 nt, synthetic construct
  source 1..20: mol_type = other RNA
gaaagagcaaggctccagga

SEQ ID NO: 2211 - RNA, 20 nt, synthetic construct
  source 1..20: mol_type = other RNA
cagacttaacaaggccttcc

SEQ ID NO: 2212 - RNA, 20 nt, synthetic construct
  source 1..20: mol_type = other RNA
ggccttgttaagtctgctcc

SEQ ID NO: 2213 - RNA, 20 nt, synthetic construct
  source 1..20: mol_type = other RNA
gccttgttaagtctgctcct

SEQ ID NO: 2214 - RNA, 20 nt, synthetic construct
  source 1..20: mol_type = other RNA
tcccaggagcagacttaaca

SEQ ID NO: 2215 - RNA, 20 nt, synthetic construct
  source 1..20: mol_type = other RNA
ggatgttacaagacagacag

SEQ ID NO: 2216 - RNA, 20 nt, synthetic construct
  source 1..20: mol_type = other RNA
tgtctgtcttgtaacatccc

SEQ ID NO: 2217 - RNA, 20 nt, synthetic construct
  source 1..20: mol_type = other RNA
gttacaagacagacagcgga

SEQ ID NO: 2218 - RNA, 20 nt, synthetic construct
  source 1..20: mol_type = other RNA
ttacaagacagacagcggac

SEQ ID NO: 2219 - RNA, 20 nt, synthetic construct
  source 1..20: mol_type = other RNA
gacttcttttggaaatgaaa

SEQ ID NO: 2220 - RNA, 20 nt, synthetic construct
  source 1..20: mol_type = other RNA
aagtatatcttgacttcttt

SEQ ID NO: 2221 - RNA, 20 nt, synthetic construct
  source 1..20: mol_type = other RNA
cttgttctgctttaaatcat

SEQ ID NO: 2222 - RNA, 20 nt, synthetic construct
  source 1..20: mol_type = other RNA
atcattttcagacatttgcg

SEQ ID NO: 2223 - RNA, 20 nt, synthetic construct
  source 1..20: mol_type = other RNA
taattttgaaatgacagttg

SEQ ID NO: 2224 - RNA, 20 nt, synthetic construct
  source 1..20: mol_type = other RNA
tatcttcatattaatattct

SEQ ID NO: 2225 - RNA, 20 nt, synthetic construct
  source 1..20: mol_type = other RNA
atattcatatgcacttcata

SEQ ID NO: 2226 - RNA, 20 nt, synthetic construct
  source 1..20: mol_type = other RNA
catattcatatgcacttcat

SEQ ID NO: 2227 - RNA, 20 nt, synthetic construct
  source 1..20: mol_type = other RNA
cacccatcgcactgtcactc

SEQ ID NO: 2228 - RNA, 20 nt, synthetic construct
  source 1..20: mol_type = other RNA
acccatcgcactgtcactca

SEQ ID NO: 2229 - RNA, 20 nt, synthetic construct
  source 1..20: mol_type = other RNA
tccctgagtgacagtgcgat

SEQ ID NO: 2230 - RNA, 20 nt, synthetic construct
  source 1..20: mol_type = other RNA
ttccctgagtgacagtgcga

SEQ ID NO: 2231 - RNA, 20 nt, synthetic construct
  source 1..20: mol_type = other RNA
ctcttaaattgcacaaatct

SEQ ID NO: 2232 - RNA, 20 nt, synthetic construct
  source 1..20: mol_type = other RNA
tttcacgttgctctccactc

SEQ ID NO: 2233 - RNA, 20 nt, synthetic construct
  source 1..20: mol_type = other RNA
gagtggagagcaacgtgaaa

SEQ ID NO: 2234 - RNA, 20 nt, synthetic construct
  source 1..20: mol_type = other RNA
agttggaagtcacacctgag

SEQ ID NO: 2235 - RNA, 20 nt, synthetic construct
  source 1..20: mol_type = other RNA
ggtttatgtgagagaggagt

SEQ ID NO: 2236 - RNA, 20 nt, synthetic construct
  source 1..20: mol_type = other RNA
aagtggggtttatgtgagag

SEQ ID NO: 2237 - RNA, 20 nt, synthetic construct
  source 1..20: mol_type = other RNA
actgcatcggcacagaagtg

SEQ ID NO: 2238 - RNA, 20 nt, synthetic construct
  source 1..20: mol_type = other RNA
gactgcatcggcacagaagt

SEQ ID NO: 2239 - RNA, 20 nt, synthetic construct
  source 1..20: mol_type = other RNA
ggactgcatcggcacagaag

SEQ ID NO: 2240 - RNA, 20 nt, synthetic construct
  source 1..20: mol_type = other RNA
agatatgtcatggactgcat

SEQ ID NO: 2241 - RNA, 20 nt, synthetic construct
  source 1..20: mol_type = other RNA
tagttagagaagatatgtca

SEQ ID NO: 2242 - RNA, 20 nt, synthetic construct
  source 1..20: mol_type = other RNA
tctctaactagacgctctga

SEQ ID NO: 2243 - RNA, 20 nt, synthetic construct
  source 1..20: mol_type = other RNA
ggaatgcctccatgatgaac

SEQ ID NO: 2244 - RNA, 20 nt, synthetic construct
  source 1..20: mol_type = other RNA
aacagaccagttcatcatgg

SEQ ID NO: 2245 - RNA, 20 nt, synthetic construct
  source 1..20: mol_type = other RNA
gggaacagaccagttcatca

SEQ ID NO: 2246 - RNA, 20 nt, synthetic construct
  source 1..20: mol_type = other RNA
tgctgaaagtattcaatgca

SEQ ID NO: 2247 - RNA, 20 nt, synthetic construct
  source 1..20: mol_type = other RNA
ttgctgaaagtattcaatgc

SEQ ID NO: 2248 - RNA, 20 nt, synthetic construct
  source 1..20: mol_type = other RNA
acaaacatattttaacctat

SEQ ID NO: 2249 - RNA, 20 nt, synthetic construct
  source 1..20: mol_type = other RNA
caaacatattttaacctata

SEQ ID NO: 2250 - RNA, 20 nt, synthetic construct
  source 1..20: mol_type = other RNA
tttaacctatagggatctaa

SEQ ID NO: 2251 - RNA, 20 nt, synthetic construct
  source 1..20: mol_type = other RNA
tcttacctttagatccctat

SEQ ID NO: 2252 - RNA, 20 nt, synthetic construct
  source 1..20: mol_type = other RNA
tttgtttgaagcttttaaaa

SEQ ID NO: 2253 - RNA, 20 nt, synthetic construct
  source 1..20: mol_type = other RNA
agtatcagtactcagagtca

SEQ ID NO: 2254 - RNA, 20 nt, synthetic construct
  source 1..20: mol_type = other RNA
ctttattgcataaaatattg

SEQ ID NO: 2255 - RNA, 20 nt, synthetic construct
  source 1..20: mol_type = other RNA
tttattgcataaaatattgt

SEQ ID NO: 2256 - RNA, 20 nt, synthetic construct
  source 1..20: mol_type = other RNA
ttgcataaaatattgtggga

SEQ ID NO: 2257 - RNA, 20 nt, synthetic construct
  source 1..20: mol_type = other RNA
tgagtagttgctacctgaat

SEQ ID NO: 2258 - RNA, 20 nt, synthetic construct
  source 1..20: mol_type = other RNA
ataggcctagtgagatcagc

SEQ ID NO: 2259 - RNA, 20 nt, synthetic construct
  source 1..20: mol_type = other RNA
gcctagtgagatcagcagga

SEQ ID NO: 2260 - RNA, 20 nt, synthetic construct
  source 1..20: mol_type = other RNA
cctagtgagatcagcaggaa

SEQ ID NO: 2261 - RNA, 20 nt, synthetic construct
  source 1..20: mol_type = other RNA
ctagtgagatcagcaggaag

SEQ ID NO: 2262 - RNA, 20 nt, synthetic construct
  source 1..20: mol_type = other RNA
cccttcctgctgatctcact

SEQ ID NO: 2263 - RNA, 20 nt, synthetic construct
  source 1..20: mol_type = other RNA
ggaaggggaaattccagcag

SEQ ID NO: 2264 - RNA, 20 nt, synthetic construct
  source 1..20: mol_type = other RNA
gaaggggaaattccagcaga

SEQ ID NO: 2265 - RNA, 20 nt, synthetic construct
  source 1..20: mol_type = other RNA
gcagagggcacatcataaag

SEQ ID NO: 2266 - RNA, 20 nt, synthetic construct
  source 1..20: mol_type = other RNA
ctttatgatgtgccctctgc

SEQ ID NO: 2267 - RNA, 20 nt, synthetic construct
  source 1..20: mol_type = other RNA
acatcataaagaggaatgaa

SEQ ID NO: 2268 - RNA, 20 nt, synthetic construct
  source 1..20: mol_type = other RNA
catcataaagaggaatgaaa

SEQ ID NO: 2269 - RNA, 20 nt, synthetic construct
  source 1..20: mol_type = other RNA
taaagaggaatgaaagggaa

SEQ ID NO: 2270 - RNA, 20 nt, synthetic construct
  source 1..20: mol_type = other RNA
aatgaaagggaatggtgtag

SEQ ID NO: 2271 - RNA, 20 nt, synthetic construct
  source 1..20: mol_type = other RNA
aaagggaatggtgtagcggc

SEQ ID NO: 2272 - RNA, 20 nt, synthetic construct
  source 1..20: mol_type = other RNA
gaatggtgtagcggcaggac

SEQ ID NO: 2273 - RNA, 20 nt, synthetic construct
  source 1..20: mol_type = other RNA
caggactggcagattcagaa

SEQ ID NO: 2274 - RNA, 20 nt, synthetic construct
  source 1..20: mol_type = other RNA
actggcagattcagaaaggc

SEQ ID NO: 2275 - RNA, 20 nt, synthetic construct
  source 1..20: mol_type = other RNA
attcagaaaggctggcgagc

SEQ ID NO: 2276 - RNA, 20 nt, synthetic construct
  source 1..20: mol_type = other RNA
ggctggcgagctggctagag

SEQ ID NO: 2277 - RNA, 20 nt, synthetic construct
  source 1..20: mol_type = other RNA
gctggcgagctggctagaga

SEQ ID NO: 2278 - RNA, 20 nt, synthetic construct
  source 1..20: mol_type = other RNA
agggctccccagacacatta

SEQ ID NO: 2279 - RNA, 20 nt, synthetic construct
  source 1..20: mol_type = other RNA
gggctccccagacacattaa

SEQ ID NO: 2280 - RNA, 20 nt, synthetic construct
  source 1..20: mol_type = other RNA
ctccccagacacattaaggg

SEQ ID NO: 2281 - RNA, 20 nt, synthetic construct
  source 1..20: mol_type = other RNA
gtccgcccttaatgtgtctg

SEQ ID NO: 2282 - RNA, 20 nt, synthetic construct
  source 1..20: mol_type = other RNA
ggtccgcccttaatgtgtct

SEQ ID NO: 2283 - RNA, 20 nt, synthetic construct
  source 1..20: mol_type = other RNA
gggtccgcccttaatgtgtc

SEQ ID NO: 2284 - RNA, 20 nt, synthetic construct
  source 1..20: mol_type = other RNA
acattaagggcggaccctga

SEQ ID NO: 2285 - RNA, 20 nt, synthetic construct
  source 1..20: mol_type = other RNA
cattaagggcggaccctgaa

SEQ ID NO: 2286 - RNA, 20 nt, synthetic construct
  source 1..20: mol_type = other RNA
ggcggaccctgaagggcacg

SEQ ID NO: 2287 - RNA, 20 nt, synthetic construct
  source 1..20: mol_type = other RNA
gcggaccctgaagggcacgt

SEQ ID NO: 2288 - RNA, 20 nt, synthetic construct
  source 1..20: mol_type = other RNA
cacggcccacgtgcccttca

SEQ ID NO: 2289 - RNA, 20 nt, synthetic construct
  source 1..20: mol_type = other RNA
gcacggcccacgtgcccttc

SEQ ID NO: 2290 - RNA, 20 nt, synthetic construct
  source 1..20: mol_type = other RNA
gggcacgtgggccgtgctac

SEQ ID NO: 2291 - RNA, 20 nt, synthetic construct
  source 1..20: mol_type = other RNA
gtgggccgtgctacaggcac

SEQ ID NO: 2292 - RNA, 20 nt, synthetic construct
  source 1..20: mol_type = other RNA
cgtgctacaggcacaggctc

SEQ ID NO: 2293 - RNA, 20 nt, synthetic construct
  source 1..20: mol_type = other RNA
cagagcctgtgcctgtagca

SEQ ID NO: 2294 - RNA, 20 nt, synthetic construct
  source 1..20: mol_type = other RNA
tacaggcacaggctctggac

SEQ ID NO: 2295 - RNA, 20 nt, synthetic construct
  source 1..20: mol_type = other RNA
acaggcacaggctctggaca

SEQ ID NO: 2296 - RNA, 20 nt, synthetic construct
  source 1..20: mol_type = other RNA
gccccagtgaagttctttaa

SEQ ID NO: 2297 - RNA, 20 nt, synthetic construct
  source 1..20: mol_type = other RNA
agtgaagttctttaaaggac

SEQ ID NO: 2298 - RNA, 20 nt, synthetic construct
  source 1..20: mol_type = other RNA
tcctttaaagaacttcactg

SEQ ID NO: 2299 - RNA, 20 nt, synthetic construct
  source 1..20: mol_type = other RNA
gtcctttaaagaacttcact

SEQ ID NO: 2300 - RNA, 20 nt, synthetic construct
  source 1..20: mol_type = other RNA
agtcctttaaagaacttcac

SEQ ID NO: 2301 - RNA, 20 nt, synthetic construct
  source 1..20: mol_type = other RNA
actctcagcagcatagaaga

SEQ ID NO: 2302 - RNA, 20 nt, synthetic construct
  source 1..20: mol_type = other RNA
gatggactgaaccaagaaga

SEQ ID NO: 2303 - RNA, 20 nt, synthetic construct
  source 1..20: mol_type = other RNA
gtatgaagttgccttcttct

SEQ ID NO: 2304 - RNA, 20 nt, synthetic construct
  source 1..20: mol_type = other RNA
tgattacgctttcagtgtat

SEQ ID NO: 2305 - RNA, 20 nt, synthetic construct
  source 1..20: mol_type = other RNA
agcgtaatcaaaaggtgatg

SEQ ID NO: 2306 - RNA, 20 nt, synthetic construct
  source 1..20: mol_type = other RNA
atgaggcctgaatcaagtag

SEQ ID NO: 2307 - RNA, 20 nt, synthetic construct
  source 1..20: mol_type = other RNA
aggcctgaatcaagtagtgg

SEQ ID NO: 2308 - RNA, 20 nt, synthetic construct
  source 1..20: mol_type = other RNA
cctgaatcaagtagtggcgg

SEQ ID NO: 2309 - RNA, 20 nt, synthetic construct
  source 1..20: mol_type = other RNA
ctgaatcaagtagtggcggt

SEQ ID NO: 2310 - RNA, 20 nt, synthetic construct
  source 1..20: mol_type = other RNA
ccaccgccactacttgattc

SEQ ID NO: 2311 - RNA, 20 nt, synthetic construct
  source 1..20: mol_type = other RNA
gaatgtaaagagtatttcca

SEQ ID NO: 2312 - RNA, 20 nt, synthetic construct
  source 1..20: mol_type = other RNA
aagctgtgatggtgctacct

SEQ ID NO: 2313 - RNA, 20 nt, synthetic construct
  source 1..20: mol_type = other RNA
ctttattagcaaagctgtga

SEQ ID NO: 2314 - RNA, 20 nt, synthetic construct
  source 1..20: mol_type = other RNA
taataaagtatacattgttt

SEQ ID NO: 2315 - RNA, 20 nt, synthetic construct
  source 1..20: mol_type = other RNA
tacattgtttaggaaacatt

SEQ ID NO: 2316 - RNA, 20 nt, synthetic construct
  source 1..20: mol_type = other RNA
agtaaactattgtttggaaa

SEQ ID NO: 2317 - RNA, 20 nt, synthetic construct
  source 1..20: mol_type = other RNA
aaggacagtaaactattgtt

SEQ ID NO: 2318 - RNA, 20 nt, synthetic construct
  source 1..20: mol_type = other RNA
gaaagacgctgatgatttca

SEQ ID NO: 2319 - RNA, 20 nt, synthetic construct
  source 1..20: mol_type = other RNA
taggatcttgaaatcatgat

SEQ ID NO: 2320 - RNA, 20 nt, synthetic construct
  source 1..20: mol_type = other RNA
ttaggatcttgaaatcatga

SEQ ID NO: 2321 - RNA, 20 nt, synthetic construct
  source 1..20: mol_type = other RNA
ttcaagatcctaaacttgac

SEQ ID NO: 2322 - RNA, 20 nt, synthetic construct
  source 1..20: mol_type = other RNA
gacattgtcctgtcaagttt

SEQ ID NO: 2323 - RNA, 20 nt, synthetic construct
  source 1..20: mol_type = other RNA
tttttcaattaggagatttg

SEQ ID NO: 2324 - RNA, 20 nt, synthetic construct
  source 1..20: mol_type = other RNA
taaagaggactttttcaatt

SEQ ID NO: 2325 - RNA, 20 nt, synthetic construct
  source 1..20: mol_type = other RNA
ctcttggggacagattaaag

SEQ ID NO: 2326 - RNA, 20 nt, synthetic construct
  source 1..20: mol_type = other RNA
cttttcattgcagactcttg

SEQ ID NO: 2327 - RNA, 20 nt, synthetic construct
  source 1..20: mol_type = other RNA
tcttttcattgcagactctt

SEQ ID NO: 2328 - RNA, 20 nt, synthetic construct
  source 1..20: mol_type = other RNA
ttcttttcattgcagactct

SEQ ID NO: 2329 - RNA, 20 nt, synthetic construct
  source 1..20: mol_type = other RNA
gagaaatgtctttacaaaat

SEQ ID NO: 2330 - RNA, 20 nt, synthetic construct
  source 1..20: mol_type = other RNA
attttgtaaagacatttctc

SEQ ID NO: 2331 - RNA, 20 nt, synthetic construct
  source 1..20: mol_type = other RNA
ataggtaaaattcattagtt

SEQ ID NO: 2332 - RNA, 20 nt, synthetic construct
  source 1..20: mol_type = other RNA
aaacagacatttttcctctt

SEQ ID NO: 2333 - RNA, 20 nt, synthetic construct
  source 1..20: mol_type = other RNA
ttttatacaagctaccaaag

SEQ ID NO: 2334 - RNA, 20 nt, synthetic construct
  source 1..20: mol_type = other RNA
atttttttttttttttgaga

SEQ ID NO: 2335 - RNA, 20 nt, synthetic construct
  source 1..20: mol_type = other RNA
atctcaaaaaaaaaaaaaaa

SEQ ID NO: 2336 - RNA, 20 nt, synthetic construct
  source 1..20: mol_type = other RNA
gagtttcgctcttgttgccc

SEQ ID NO: 2337 - RNA, 20 nt, synthetic construct
  source 1..20: mol_type = other RNA
ttcgctcttgttgcccaggc

SEQ ID NO: 2338 - RNA, 20 nt, synthetic construct
  source 1..20: mol_type = other RNA
ttgcccaggctggagtgcaa

SEQ ID NO: 2339 - RNA, 20 nt, synthetic construct
  source 1..20: mol_type = other RNA
gcaccattgcactccagcct

SEQ ID NO: 2340 - RNA, 20 nt, synthetic construct
  source 1..20: mol_type = other RNA
cgcaccattgcactccagcc

SEQ ID NO: 2341 - RNA, 20 nt, synthetic construct
  source 1..20: mol_type = other RNA
tcaccacaacctccacctcc

SEQ ID NO: 2342 - RNA, 20 nt, synthetic construct
  source 1..20: mol_type = other RNA
caccacaacctccacctcct

SEQ ID NO: 2343 - RNA, 20 nt, synthetic construct
  source 1..20: mol_type = other RNA
aacccaggaggtggaggttg

SEQ ID NO: 2344 - RNA, 20 nt, synthetic construct
  source 1..20: mol_type = other RNA
tgcttgaacccaggaggtgg

SEQ ID NO: 2345 - RNA, 20 nt, synthetic construct
  source 1..20: mol_type = other RNA
aattgcttgaacccaggagg

SEQ ID NO: 2346 - RNA, 20 nt, synthetic construct
  source 1..20: mol_type = other RNA
gagaattgcttgaacccagg

SEQ ID NO: 2347 - RNA, 20 nt, synthetic construct
  source 1..20: mol_type = other RNA
caggagaattgcttgaaccc

SEQ ID NO: 2348 - RNA, 20 nt, synthetic construct
  source 1..20: mol_type = other RNA
gcctcagcctcctgagtagc

SEQ ID NO: 2349 - RNA, 20 nt, synthetic construct
  source 1..20: mol_type = other RNA
cctcagcctcctgagtagct

SEQ ID NO: 2350 - RNA, 20 nt, synthetic construct
  source 1..20: mol_type = other RNA
gctactcaggaggctgaggc

SEQ ID NO: 2351 - RNA, 20 nt, synthetic construct
  source 1..20: mol_type = other RNA
cccagctactcaggaggctg

SEQ ID NO: 2352 - RNA, 20 nt, synthetic construct
  source 1..20: mol_type = other RNA
tcctgagtagctgggattac

SEQ ID NO: 2353 - RNA, 20 nt, synthetic construct
  source 1..20: mol_type = other RNA
tgtaatcccagctactcagg

SEQ ID NO: 2354 - RNA, 20 nt, synthetic construct
  source 1..20: mol_type = other RNA
gcctgtaatcccagctactc

SEQ ID NO: 2355 - RNA, 20 nt, synthetic construct
  source 1..20: mol_type = other RNA
acaaaattagctgggcgtgg

SEQ ID NO: 2356 - RNA, 20 nt, synthetic construct
  source 1..20: mol_type = other RNA
aatacaaaattagctgggcg

SEQ ID NO: 2357 - RNA, 20 nt, synthetic construct
  source 1..20: mol_type = other RNA
ctaaaaatacaaaattagct

SEQ ID NO: 2358 - RNA, 20 nt, synthetic construct
  source 1..20: mol_type = other RNA
gctaaaaatacaaaattagc

SEQ ID NO: 2359 - RNA, 20 nt, synthetic construct
  source 1..20: mol_type = other RNA
ttttgtatttttagcagaga

SEQ ID NO: 2360 - RNA, 20 nt, synthetic construct
  source 1..20: mol_type = other RNA
tttgtatttttagcagagac

SEQ ID NO: 2361 - RNA, 20 nt, synthetic construct
  source 1..20: mol_type = other RNA
ttgtatttttagcagagacg

SEQ ID NO: 2362 - RNA, 20 nt, synthetic construct
  source 1..20: mol_type = other RNA
gagacggggtttctccatgt

SEQ ID NO: 2363 - RNA, 20 nt, synthetic construct
  source 1..20: mol_type = other RNA
ggggtttctccatgttggtc

SEQ ID NO: 2364 - RNA, 20 nt, synthetic construct
  source 1..20: mol_type = other RNA
tttctccatgttggtcaggc

SEQ ID NO: 2365 - RNA, 20 nt, synthetic construct
  source 1..20: mol_type = other RNA
caagaccagcctgaccaaca

SEQ ID NO: 2366 - RNA, 20 nt, synthetic construct
  source 1..20: mol_type = other RNA
ggtcttgaactctcgacctc

SEQ ID NO: 2367 - RNA, 20 nt, synthetic construct
  source 1..20: mol_type = other RNA
ctcaggtgatccacctgcct

SEQ ID NO: 2368 - RNA, 20 nt, synthetic construct
  source 1..20: mol_type = other RNA
cgaggcaggtggatcacctg

SEQ ID NO: 2369 - RNA, 20 nt, synthetic construct
  source 1..20: mol_type = other RNA
ctttgggaggccgaggcagg

SEQ ID NO: 2370 - RNA, 20 nt, synthetic construct
  source 1..20: mol_type = other RNA
gcctcggcctcccaaagtgt

SEQ ID NO: 2371 - RNA, 20 nt, synthetic construct
  source 1..20: mol_type = other RNA
cctcggcctcccaaagtgtt

SEQ ID NO: 2372 - RNA, 20 nt, synthetic construct
  source 1..20: mol_type = other RNA
acactttgggaggccgaggc

SEQ ID NO: 2373 - RNA, 20 nt, synthetic construct
  source 1..20: mol_type = other RNA
cccaacactttgggaggccg

SEQ ID NO: 2374 - RNA, 20 nt, synthetic construct
  source 1..20: mol_type = other RNA
tcccaaagtgttgggattac

SEQ ID NO: 2375 - RNA, 20 nt, synthetic construct
  source 1..20: mol_type = other RNA
tgtaatcccaacactttggg

SEQ ID NO: 2376 - RNA, 20 nt, synthetic construct
  source 1..20: mol_type = other RNA
tcctgtaatcccaacacttt

SEQ ID NO: 2377 - RNA, 20 nt, synthetic construct
  source 1..20: mol_type = other RNA
ctcctgtaatcccaacactt

SEQ ID NO: 2378 - RNA, 20 nt, synthetic construct
  source 1..20: mol_type = other RNA
gggattacaggagtgagcca

SEQ ID NO: 2379 - RNA, 20 nt, synthetic construct
  source 1..20: mol_type = other RNA
tgcaatactgctgagcgccg

SEQ ID NO: 2380 - RNA, 20 nt, synthetic construct
  source 1..20: mol_type = other RNA
agtctgagtttcaaagaaaa

SEQ ID NO: 2381 - RNA, 20 nt, synthetic construct
  source 1..20: mol_type = other RNA
aactcagactctccgcttct

SEQ ID NO: 2382 - RNA, 20 nt, synthetic construct
  source 1..20: mol_type = other RNA
ggctctaactctcctagaag

SEQ ID NO: 2383 - RNA, 20 nt, synthetic construct
  source 1..20: mol_type = other RNA
ttagagcctaaacaaattga

SEQ ID NO: 2384 - RNA, 20 nt, synthetic construct
  source 1..20: mol_type = other RNA
gagcctaaacaaattgaagg

SEQ ID NO: 2385 - RNA, 20 nt, synthetic construct
  source 1..20: mol_type = other RNA
cctaaacaaattgaaggtgg

SEQ ID NO: 2386 - RNA, 20 nt, synthetic construct
  source 1..20: mol_type = other RNA
ctaaacaaattgaaggtgga

SEQ ID NO: 2387 - RNA, 20 nt, synthetic construct
  source 1..20: mol_type = other RNA
cctccaccttcaatttgttt

SEQ ID NO: 2388 - RNA, 20 nt, synthetic construct
  source 1..20: mol_type = other RNA
aattgaaggtggagggactt

SEQ ID NO: 2389 - RNA, 20 nt, synthetic construct
  source 1..20: mol_type = other RNA
attgaaggtggagggactta

SEQ ID NO: 2390 - RNA, 20 nt, synthetic construct
  source 1..20: mol_type = other RNA
ttgaaggtggagggacttag

SEQ ID NO: 2391 - RNA, 20 nt, synthetic construct
  source 1..20: mol_type = other RNA
ttaactttcatcacatccaa

SEQ ID NO: 2392 - RNA, 20 nt, synthetic construct
  source 1..20: mol_type = other RNA
catggtgtctcatgggcctt

SEQ ID NO: 2393 - RNA, 20 nt, synthetic construct
  source 1..20: mol_type = other RNA
gagacaccatgcaaacaatg

SEQ ID NO: 2394 - RNA, 20 nt, synthetic construct
  source 1..20: mol_type = other RNA
attgtttgcatggtgtctca

SEQ ID NO: 2395 - RNA, 20 nt, synthetic construct
  source 1..20: mol_type = other RNA
tttggtccgcattgtttgca

SEQ ID NO: 2396 - RNA, 20 nt, synthetic construct
  source 1..20: mol_type = other RNA
tgcggaccaaatatctatat

SEQ ID NO: 2397 - RNA, 20 nt, synthetic construct
  source 1..20: mol_type = other RNA
atatcaccaatatagatatt

SEQ ID NO: 2398 - RNA, 20 nt, synthetic construct
  source 1..20: mol_type = other RNA
atgctaagaaaaaagagtaa

SEQ ID NO: 2399 - RNA, 20 nt, synthetic construct
  source 1..20: mol_type = other RNA
tgctaagaaaaaagagtaac

SEQ ID NO: 2400 - RNA, 20 nt, synthetic construct
  source 1..20: mol_type = other RNA
agtaacgggactcacagcgc

SEQ ID NO: 2401 - RNA, 20 nt, synthetic construct
  source 1..20: mol_type = other RNA
gtaacgggactcacagcgct

SEQ ID NO: 2402 - RNA, 20 nt, synthetic construct
  source 1..20: mol_type = other RNA
taacgggactcacagcgctg

SEQ ID NO: 2403 - RNA, 20 nt, synthetic construct
  source 1..20: mol_type = other RNA
ggactcacagcgctggggag

SEQ ID NO: 2404 - RNA, 20 nt, synthetic construct
  source 1..20: mol_type = other RNA
gactcacagcgctggggaga

SEQ ID NO: 2405 - RNA, 20 nt, synthetic construct
  source 1..20: mol_type = other RNA
actcacagcgctggggagag

SEQ ID NO: 2406 - RNA, 20 nt, synthetic construct
  source 1..20: mol_type = other RNA
acagcgctggggagaggggc

SEQ ID NO: 2407 - RNA, 20 nt, synthetic construct
  source 1..20: mol_type = other RNA
ggcaggttgcaattctaaac

SEQ ID NO: 2408 - RNA, 20 nt, synthetic construct
  source 1..20: mol_type = other RNA
gcaggttgcaattctaaaca

SEQ ID NO: 2409 - RNA, 20 nt, synthetic construct
  source 1..20: mol_type = other RNA
ggttgcaattctaaacaggg

SEQ ID NO: 2410 - RNA, 20 nt, synthetic construct
  source 1..20: mol_type = other RNA
caattctaaacagggtggtc

SEQ ID NO: 2411 - RNA, 20 nt, synthetic construct
  source 1..20: mol_type = other RNA
gtagtgaaaaggagggcttg

SEQ ID NO: 2412 - RNA, 20 nt, synthetic construct
  source 1..20: mol_type = other RNA
tgtagtgaaaaggagggctt

SEQ ID NO: 2413 - RNA, 20 nt, synthetic construct
  source 1..20: mol_type = other RNA
atgtagtgaaaaggagggct

SEQ ID NO: 2414 - RNA, 20 nt, synthetic construct
  source 1..20: mol_type = other RNA
gcaggatgtagtgaaaagga

SEQ ID NO: 2415 - RNA, 20 nt, synthetic construct
  source 1..20: mol_type = other RNA
ggcaggatgtagtgaaaagg

SEQ ID NO: 2416 - RNA, 20 nt, synthetic construct
  source 1..20: mol_type = other RNA
ggaggcaggatgtagtgaaa

SEQ ID NO: 2417 - RNA, 20 nt, synthetic construct
  source 1..20: mol_type = other RNA
tttggtttgttttaggaggc

SEQ ID NO: 2418 - RNA, 20 nt, synthetic construct
  source 1..20: mol_type = other RNA
attttttggtttgttttagg

SEQ ID NO: 2419 - RNA, 20 nt, synthetic construct
  source 1..20: mol_type = other RNA
tgtattttttggtttgtttt

SEQ ID NO: 2420 - RNA, 20 nt, synthetic construct
  source 1..20: mol_type = other RNA
ttgtgtgcatgtgtattttt

SEQ ID NO: 2421 - RNA, 20 nt, synthetic construct
  source 1..20: mol_type = other RNA
caaacccacaagtacttaca

SEQ ID NO: 2422 - RNA, 20 nt, synthetic construct
  source 1..20: mol_type = other RNA
aaacccacaagtacttacat

SEQ ID NO: 2423 - RNA, 20 nt, synthetic construct
  source 1..20: mol_type = other RNA
aagcccatgtaagtacttgt

SEQ ID NO: 2424 - RNA, 20 nt, synthetic construct
  source 1..20: mol_type = other RNA
taagcccatgtaagtacttg

SEQ ID NO: 2425 - RNA, 20 nt, synthetic construct
  source 1..20: mol_type = other RNA
aatatatttttgttatttta

SEQ ID NO: 2426 - RNA, 20 nt, synthetic construct
  source 1..20: mol_type = other RNA
ttgctgtggagaatttaaga

SEQ ID NO: 2427 - RNA, 20 nt, synthetic construct
  source 1..20: mol_type = other RNA
tttgctgtggagaatttaag

SEQ ID NO: 2428 - RNA, 20 nt, synthetic construct
  source 1..20: mol_type = other RNA
tgggaagataagttttgctg

SEQ ID NO: 2429 - RNA, 20 nt, synthetic construct
  source 1..20: mol_type = other RNA
catgttattttacgctggct

SEQ ID NO: 2430 - RNA, 20 nt, synthetic construct
  source 1..20: mol_type = other RNA
tcatgttattttacgctggc

SEQ ID NO: 2431 - RNA, 20 nt, synthetic construct
  source 1..20: mol_type = other RNA
tgcttcatgttattttacgc

SEQ ID NO: 2432 - RNA, 20 nt, synthetic construct
  source 1..20: mol_type = other RNA
ttatgatatgccaagtacta

SEQ ID NO: 2433 - RNA, 20 nt, synthetic construct
  source 1..20: mol_type = other RNA
aatgtgctttccatagtact

SEQ ID NO: 2434 - RNA, 20 nt, synthetic construct
  source 1..20: mol_type = other RNA
tttaatcctcacaatactaa

SEQ ID NO: 2435 - RNA, 20 nt, synthetic construct
  source 1..20: mol_type = other RNA
tcgtttccattagtattgtg

SEQ ID NO: 2436 - RNA, 20 nt, synthetic construct
  source 1..20: mol_type = other RNA
tcttccccattatatctgtg

SEQ ID NO: 2437 - RNA, 20 nt, synthetic construct
  source 1..20: mol_type = other RNA
cttccccattatatctgtga

SEQ ID NO: 2438 - RNA, 20 nt, synthetic construct
  source 1..20: mol_type = other RNA
catccctcacagatataatg

SEQ ID NO: 2439 - RNA, 20 nt, synthetic construct
  source 1..20: mol_type = other RNA
tcatccctcacagatataat

SEQ ID NO: 2440 - RNA, 20 nt, synthetic construct
  source 1..20: mol_type = other RNA
ttcatccctcacagatataa

SEQ ID NO: 2441 - RNA, 20 nt, synthetic construct
  source 1..20: mol_type = other RNA
gagggatgaaaggctttcaa

SEQ ID NO: 2442 - RNA, 20 nt, synthetic construct
  source 1..20: mol_type = other RNA
actagctatgggatctttgg

SEQ ID NO: 2443 - RNA, 20 nt, synthetic construct
  source 1..20: mol_type = other RNA
aagatcccatagctagtaag

SEQ ID NO: 2444 - RNA, 20 nt, synthetic construct
  source 1..20: mol_type = other RNA
cttactagctatgggatctt

SEQ ID NO: 2445 - RNA, 20 nt, synthetic construct
  source 1..20: mol_type = other RNA
gactgccacttactagctat

SEQ ID NO: 2446 - RNA, 20 nt, synthetic construct
  source 1..20: mol_type = other RNA
ggactgccacttactagcta

SEQ ID NO: 2447 - RNA, 20 nt, synthetic construct
  source 1..20: mol_type = other RNA
gcagtcccagcattgaacca

SEQ ID NO: 2448 - RNA, 20 nt, synthetic construct
  source 1..20: mol_type = other RNA
aaggaccttggttcaatgct

SEQ ID NO: 2449 - RNA, 20 nt, synthetic construct
  source 1..20: mol_type = other RNA
gaaggaccttggttcaatgc

SEQ ID NO: 2450 - RNA, 20 nt, synthetic construct
  source 1..20: mol_type = other RNA
ctttggcatctgaaggacct

SEQ ID NO: 2451 - RNA, 20 nt, synthetic construct
  source 1..20: mol_type = other RNA
gcacagactttggcatctga

SEQ ID NO: 2452 - RNA, 20 nt, synthetic construct
  source 1..20: mol_type = other RNA
cagatctagagcacagactt

SEQ ID NO: 2453 - RNA, 20 nt, synthetic construct
  source 1..20: mol_type = other RNA
ctgtttacttactgctaatt

SEQ ID NO: 2454 - RNA, 20 nt, synthetic construct
  source 1..20: mol_type = other RNA
agtgtttgatgcttgcttgt

SEQ ID NO: 2455 - RNA, 20 nt, synthetic construct
  source 1..20: mol_type = other RNA
atgaagcagaattaatgcaa

SEQ ID NO: 2456 - RNA, 20 nt, synthetic construct
  source 1..20: mol_type = other RNA
aagcagaattaatgcaatgg

SEQ ID NO: 2457 - RNA, 20 nt, synthetic construct
  source 1..20: mol_type = other RNA
taatgcaatggaggtatcta

SEQ ID NO: 2458 - RNA, 20 nt, synthetic construct
  source 1..20: mol_type = other RNA
gtcagaatttgaatatgatg

SEQ ID NO: 2459 - RNA, 20 nt, synthetic construct
  source 1..20: mol_type = other RNA
cacagcatctacctaaattt

SEQ ID NO: 2460 - RNA, 20 nt, synthetic construct
  source 1..20: mol_type = other RNA
aggtagaaactccaaaattt

SEQ ID NO: 2461 - RNA, 20 nt, synthetic construct
  source 1..20: mol_type = other RNA
atgaagaaataaatattttc

SEQ ID NO: 2462 - RNA, 20 nt, synthetic construct
  source 1..20: mol_type = other RNA
taaaatttgaggatatttct

SEQ ID NO: 2463 - RNA, 20 nt, synthetic construct
  source 1..20: mol_type = other RNA
ataaaatttgaggatatttc

SEQ ID NO: 2464 - RNA, 20 nt, synthetic construct
  source 1..20: mol_type = other RNA
catgatagaaataaaatttg

SEQ ID NO: 2465 - RNA, 20 nt, synthetic construct
  source 1..20: mol_type = other RNA
tagaaataatttttttttta

SEQ ID NO: 2466 - RNA, 20 nt, synthetic construct
  source 1..20: mol_type = other RNA
taaatgttcagcaacaagcc

SEQ ID NO: 2467 - RNA, 20 nt, synthetic construct
  source 1..20: mol_type = other RNA
ggcttgttgctgaacattta

SEQ ID NO: 2468 - RNA, 20 nt, synthetic construct
  source 1..20: mol_type = other RNA
cagcaacaagcctggcgcag

SEQ ID NO: 2469 - RNA, 20 nt, synthetic construct
  source 1..20: mol_type = other RNA
caggcgttagccactgcgcc

SEQ ID NO: 2470 - RNA, 20 nt, synthetic construct
  source 1..20: mol_type = other RNA
cgcctgtaatcccaacactt

SEQ ID NO: 2471 - RNA, 20 nt, synthetic construct
  source 1..20: mol_type = other RNA
gcctgtaatcccaacacttt

SEQ ID NO: 2472 - RNA, 20 nt, synthetic construct
  source 1..20: mol_type = other RNA
tgtaatcccaacactttggg

SEQ ID NO: 2473 - RNA, 20 nt, synthetic construct
  source 1..20: mol_type = other RNA
tcccaaagtgttgggattac

SEQ ID NO: 2474 - RNA, 20 nt, synthetic construct
  source 1..20: mol_type = other RNA
cccaacactttgggaggccg

SEQ ID NO: 2475 - RNA, 20 nt, synthetic construct
  source 1..20: mol_type = other RNA
acactttgggaggccgaggc

SEQ ID NO: 2476 - RNA, 20 nt, synthetic construct
  source 1..20: mol_type = other RNA
cctcggcctcccaaagtgtt

SEQ ID NO: 2477 - RNA, 20 nt, synthetic construct
  source 1..20: mol_type = other RNA
gcctcggcctcccaaagtgt

SEQ ID NO: 2478 - RNA, 20 nt, synthetic construct
  source 1..20: mol_type = other RNA
ctttgggaggccgaggcagg

SEQ ID NO: 2479 - RNA, 20 nt, synthetic construct
  source 1..20: mol_type = other RNA
cgaggcaggcggattccctg

SEQ ID NO: 2480 - RNA, 20 nt, synthetic construct
  source 1..20: mol_type = other RNA
ctcagggaatccgcctgcct

SEQ ID NO: 2481 - RNA, 20 nt, synthetic construct
  source 1..20: mol_type = other RNA
caggcggattccctgaggtc

SEQ ID NO: 2482 - RNA, 20 nt, synthetic construct
  source 1..20: mol_type = other RNA
gtctcaaactcctgacctca

SEQ ID NO: 2483 - RNA, 20 nt, synthetic construct
  source 1..20: mol_type = other RNA
cgtctcaaactcctgacctc

SEQ ID NO: 2484 - RNA, 20 nt, synthetic construct
  source 1..20: mol_type = other RNA
tcaggagtttgagacgagcc

SEQ ID NO: 2485 - RNA, 20 nt, synthetic construct
  source 1..20: mol_type = other RNA
gggttttcacaatgttggcc

SEQ ID NO: 2486 - RNA, 20 nt, synthetic construct
  source 1..20: mol_type = other RNA
gagctgggttttcacaatgt

SEQ ID NO: 2487 - RNA, 20 nt, synthetic construct
  source 1..20: mol_type = other RNA
tttgtatttttaatagagct

SEQ ID NO: 2488 - RNA, 20 nt, synthetic construct
  source 1..20: mol_type = other RNA
ttttgtatttttaatagagc

SEQ ID NO: 2489 - RNA, 20 nt, synthetic construct
  source 1..20: mol_type = other RNA
ctattaaaaatacaaaaatt

SEQ ID NO: 2490 - RNA, 20 nt, synthetic construct
  source 1..20: mol_type = other RNA
aaaaatacaaaaatttggcc

SEQ ID NO: 2491 - RNA, 20 nt, synthetic construct
  source 1..20: mol_type = other RNA
tacaaaaatttggccaggtg

SEQ ID NO: 2492 - RNA, 20 nt, synthetic construct
  source 1..20: mol_type = other RNA
aaaaatttggccaggtgtgg

SEQ ID NO: 2493 - RNA, 20 nt, synthetic construct
  source 1..20: mol_type = other RNA
caggtgtgagccaccacacc

SEQ ID NO: 2494 - RNA, 20 nt, synthetic construct
  source 1..20: mol_type = other RNA
cacctgtaataccagcgctt

SEQ ID NO: 2495 - RNA, 20 nt, synthetic construct
  source 1..20: mol_type = other RNA
acctgtaataccagcgcttt

SEQ ID NO: 2496 - RNA, 20 nt, synthetic construct
  source 1..20: mol_type = other RNA
tgtaataccagcgctttggg

SEQ ID NO: 2497 - RNA, 20 nt, synthetic construct
  source 1..20: mol_type = other RNA
tcccaaagcgctggtattac

SEQ ID NO: 2498 - RNA, 20 nt, synthetic construct
  source 1..20: mol_type = other RNA
accagcgctttgggaggccg

SEQ ID NO: 2499 - RNA, 20 nt, synthetic construct
  source 1..20: mol_type = other RNA
agcgctttgggaggccgagg

SEQ ID NO: 2500 - RNA, 20 nt, synthetic construct
  source 1..20: mol_type = other RNA
gcgctttgggaggccgaggc

SEQ ID NO: 2501 - RNA, 20 nt, synthetic construct
  source 1..20: mol_type = other RNA
cgctttgggaggccgaggcg

SEQ ID NO: 2502 - RNA, 20 nt, synthetic construct
  source 1..20: mol_type = other RNA
gcctcggcctcccaaagcgc

SEQ ID NO: 2503 - RNA, 20 nt, synthetic construct
  source 1..20: mol_type = other RNA
ccgaggcggggaatcacctg

SEQ ID NO: 2504 - RNA, 20 nt, synthetic construct
  source 1..20: mol_type = other RNA
cctcaggtgattccccgcct

SEQ ID NO: 2505 - RNA, 20 nt, synthetic construct
  source 1..20: mol_type = other RNA
ggtctcaaactcctgacctc

SEQ ID NO: 2506 - RNA, 20 nt, synthetic construct
  source 1..20: mol_type = other RNA
tcaggagtttgagaccaacc

SEQ ID NO: 2507 - RNA, 20 nt, synthetic construct
  source 1..20: mol_type = other RNA
tttcgctttgttggccaggt

SEQ ID NO: 2508 - RNA, 20 nt, synthetic construct
  source 1..20: mol_type = other RNA
ggggtttcgctttgttggcc

SEQ ID NO: 2509 - RNA, 20 nt, synthetic construct
  source 1..20: mol_type = other RNA
gagacggggtttcgctttgt

SEQ ID NO: 2510 - RNA, 20 nt, synthetic construct
  source 1..20: mol_type = other RNA
ttgtatatttagtagagacg

SEQ ID NO: 2511 - RNA, 20 nt, synthetic construct
  source 1..20: mol_type = other RNA
tttgtatatttagtagagac

SEQ ID NO: 2512 - RNA, 20 nt, synthetic construct
  source 1..20: mol_type = other RNA
ttttgtatatttagtagaga

SEQ ID NO: 2513 - RNA, 20 nt, synthetic construct
  source 1..20: mol_type = other RNA
aaatatacaaaaaatcagct

SEQ ID NO: 2514 - RNA, 20 nt, synthetic construct
  source 1..20: mol_type = other RNA
tacaaaaaatcagctaggcg

SEQ ID NO: 2515 - RNA, 20 nt, synthetic construct
  source 1..20: mol_type = other RNA
aaatcagctaggcgtggtga

SEQ ID NO: 2516 - RNA, 20 nt, synthetic construct
  source 1..20: mol_type = other RNA
aatcagctaggcgtggtgat

SEQ ID NO: 2517 - RNA, 20 nt, synthetic construct
  source 1..20: mol_type = other RNA
tgcctgtaatcccagctact

SEQ ID NO: 2518 - RNA, 20 nt, synthetic construct
  source 1..20: mol_type = other RNA
gcctgtaatcccagctactc

SEQ ID NO: 2519 - RNA, 20 nt, synthetic construct
  source 1..20: mol_type = other RNA
tgtaatcccagctactcggg

SEQ ID NO: 2520 - RNA, 20 nt, synthetic construct
  source 1..20: mol_type = other RNA
tcccgagtagctgggattac

SEQ ID NO: 2521 - RNA, 20 nt, synthetic construct
  source 1..20: mol_type = other RNA
cccagctactcgggaggctg

SEQ ID NO: 2522 - RNA, 20 nt, synthetic construct
  source 1..20: mol_type = other RNA
cctcagcctcccgagtagct

SEQ ID NO: 2523 - RNA, 20 nt, synthetic construct
  source 1..20: mol_type = other RNA
gcctcagcctcccgagtagc

SEQ ID NO: 2524 - RNA, 20 nt, synthetic construct
  source 1..20: mol_type = other RNA
gcagaagaattgcttgaacc

SEQ ID NO: 2525 - RNA, 20 nt, synthetic construct
  source 1..20: mol_type = other RNA
cagaagaattgcttgaaccc

SEQ ID NO: 2526 - RNA, 20 nt, synthetic construct
  source 1..20: mol_type = other RNA
aagaattgcttgaacccggg

SEQ ID NO: 2527 - RNA, 20 nt, synthetic construct
  source 1..20: mol_type = other RNA
aattgcttgaacccgggagg

SEQ ID NO: 2528 - RNA, 20 nt, synthetic construct
  source 1..20: mol_type = other RNA
tgcttgaacccgggaggtgg

SEQ ID NO: 2529 - RNA, 20 nt, synthetic construct
  source 1..20: mol_type = other RNA
cactgtaacctccacctccc

SEQ ID NO: 2530 - RNA, 20 nt, synthetic construct
  source 1..20: mol_type = other RNA
tcactgtaacctccacctcc

SEQ ID NO: 2531 - RNA, 20 nt, synthetic construct
  source 1..20: mol_type = other RNA
ggagtgcaatggcacgatct

SEQ ID NO: 2532 - RNA, 20 nt, synthetic construct
  source 1..20: mol_type = other RNA
cgtgccattgcactccagtc

SEQ ID NO: 2533 - RNA, 20 nt, synthetic construct
  source 1..20: mol_type = other RNA
gtgccattgcactccagtct

SEQ ID NO: 2534 - RNA, 20 nt, synthetic construct
  source 1..20: mol_type = other RNA
tcgcccagactggagtgcaa

SEQ ID NO: 2535 - RNA, 20 nt, synthetic construct
  source 1..20: mol_type = other RNA
tctcactctgtcgcccagac

SEQ ID NO: 2536 - RNA, 20 nt, synthetic construct
  source 1..20: mol_type = other RNA
cccaaaaaaatacaaaaatt

SEQ ID NO: 2537 - RNA, 20 nt, synthetic construct
  source 1..20: mol_type = other RNA
ctaatttttgtatttttttg

SEQ ID NO: 2538 - RNA, 20 nt, synthetic construct
  source 1..20: mol_type = other RNA
cctaatttttgtattttttt

SEQ ID NO: 2539 - RNA, 20 nt, synthetic construct
  source 1..20: mol_type = other RNA
gcctaatttttgtatttttt

SEQ ID NO: 2540 - RNA, 20 nt, synthetic construct
  source 1..20: mol_type = other RNA
tacaaaaattaggctgtgcg

SEQ ID NO: 2541 - RNA, 20 nt, synthetic construct
  source 1..20: mol_type = other RNA
aaaaattaggctgtgcgcgg

SEQ ID NO: 2542 - RNA, 20 nt, synthetic construct
  source 1..20: mol_type = other RNA
tgcctgtaatcccagcactt

SEQ ID NO: 2543 - RNA, 20 nt, synthetic construct
  source 1..20: mol_type = other RNA
gcctgtaatcccagcacttt

SEQ ID NO: 2544 - RNA, 20 nt, synthetic construct
  source 1..20: mol_type = other RNA
tgtaatcccagcactttggg

SEQ ID NO: 2545 - RNA, 20 nt, synthetic construct
  source 1..20: mol_type = other RNA
tcccaaagtgctgggattac

SEQ ID NO: 2546 - RNA, 20 nt, synthetic construct
  source 1..20: mol_type = other RNA
cccagcactttgggaggccg

SEQ ID NO: 2547 - RNA, 20 nt, synthetic construct
  source 1..20: mol_type = other RNA
agcactttgggaggccgagg

SEQ ID NO: 2548 - RNA, 20 nt, synthetic construct
  source 1..20: mol_type = other RNA
gcactttgggaggccgaggt

SEQ ID NO: 2549 - RNA, 20 nt, synthetic construct
  source 1..20: mol_type = other RNA
cctcggcctcccaaagtgct

SEQ ID NO: 2550 - RNA, 20 nt, synthetic construct
  source 1..20: mol_type = other RNA
acctcggcctcccaaagtgc

SEQ ID NO: 2551 - RNA, 20 nt, synthetic construct
  source 1..20: mol_type = other RNA
ctttgggaggccgaggtggg

SEQ ID NO: 2552 - RNA, 20 nt, synthetic construct
  source 1..20: mol_type = other RNA
gccgaggtgggtggatcacg

SEQ ID NO: 2553 - RNA, 20 nt, synthetic construct
  source 1..20: mol_type = other RNA
ggtgggtggatcacgaggtc

SEQ ID NO: 2554 - RNA, 20 nt, synthetic construct
  source 1..20: mol_type = other RNA
acctcgtgatccacccacct

SEQ ID NO: 2555 - RNA, 20 nt, synthetic construct
  source 1..20: mol_type = other RNA
tcaggagttcaagaccagcc

SEQ ID NO: 2556 - RNA, 20 nt, synthetic construct
  source 1..20: mol_type = other RNA
agttcaagaccagcctggcc

SEQ ID NO: 2557 - RNA, 20 nt, synthetic construct
  source 1..20: mol_type = other RNA
caagaccagcctggccagga

SEQ ID NO: 2558 - RNA, 20 nt, synthetic construct
  source 1..20: mol_type = other RNA
tttcaccatcctggccaggc

SEQ ID NO: 2559 - RNA, 20 nt, synthetic construct
  source 1..20: mol_type = other RNA
gaggtttcaccatcctggcc

SEQ ID NO: 2560 - RNA, 20 nt, synthetic construct
  source 1..20: mol_type = other RNA
gagacgaggtttcaccatcc

SEQ ID NO: 2561 - RNA, 20 nt, synthetic construct
  source 1..20: mol_type = other RNA
ttgtagtttcagtagagacg

SEQ ID NO: 2562 - RNA, 20 nt, synthetic construct
  source 1..20: mol_type = other RNA
tgaaactacaaaaattagcc

SEQ ID NO: 2563 - RNA, 20 nt, synthetic construct
  source 1..20: mol_type = other RNA
caaaaattagccaggcgcga

SEQ ID NO: 2564 - RNA, 20 nt, synthetic construct
  source 1..20: mol_type = other RNA
aattagccaggcgcgatggc

SEQ ID NO: 2565 - RNA, 20 nt, synthetic construct
  source 1..20: mol_type = other RNA
caggtgcctgccatcgcgcc

SEQ ID NO: 2566 - RNA, 20 nt, synthetic construct
  source 1..20: mol_type = other RNA
cacctgtaatcccagctact

SEQ ID NO: 2567 - RNA, 20 nt, synthetic construct
  source 1..20: mol_type = other RNA
acctgtaatcccagctactc

SEQ ID NO: 2568 - RNA, 20 nt, synthetic construct
  source 1..20: mol_type = other RNA
tgtaatcccagctactcggg

SEQ ID NO: 2569 - RNA, 20 nt, synthetic construct
  source 1..20: mol_type = other RNA
tcccgagtagctgggattac

SEQ ID NO: 2570 - RNA, 20 nt, synthetic construct
  source 1..20: mol_type = other RNA
cccagctactcgggaggctg

SEQ ID NO: 2571 - RNA, 20 nt, synthetic construct
  source 1..20: mol_type = other RNA
gctactcgggaggctgaggc

SEQ ID NO: 2572 - RNA, 20 nt, synthetic construct
  source 1..20: mol_type = other RNA
cctcagcctcccgagtagct

SEQ ID NO: 2573 - RNA, 20 nt, synthetic construct
  source 1..20: mol_type = other RNA
gcctcagcctcccgagtagc

SEQ ID NO: 2574 - RNA, 20 nt, synthetic construct
  source 1..20: mol_type = other RNA
gcaggagaatcgcttgaaac

SEQ ID NO: 2575 - RNA, 20 nt, synthetic construct
  source 1..20: mol_type = other RNA
caggagaatcgcttgaaacc

SEQ ID NO: 2576 - RNA, 20 nt, synthetic construct
  source 1..20: mol_type = other RNA
gagaatcgcttgaaaccggg

SEQ ID NO: 2577 - RNA, 20 nt, synthetic construct
  source 1..20: mol_type = other RNA
cgcttgaaaccgggtggctg

SEQ ID NO: 2578 - RNA, 20 nt, synthetic construct
  source 1..20: mol_type = other RNA
tcactgcaacctcagccacc

SEQ ID NO: 2579 - RNA, 20 nt, synthetic construct
  source 1..20: mol_type = other RNA
gctgaggttgcagtgagccg

SEQ ID NO: 2580 - RNA, 20 nt, synthetic construct
  source 1..20: mol_type = other RNA
agagtacagtggtacgacct

SEQ ID NO: 2581 - RNA, 20 nt, synthetic construct
  source 1..20: mol_type = other RNA
cgtaccactgtactctagcc

SEQ ID NO: 2582 - RNA, 20 nt, synthetic construct
  source 1..20: mol_type = other RNA
gtaccactgtactctagcct

SEQ ID NO: 2583 - RNA, 20 nt, synthetic construct
  source 1..20: mol_type = other RNA
tcacccaggctagagtacag

SEQ ID NO: 2584 - RNA, 20 nt, synthetic construct
  source 1..20: mol_type = other RNA
ctagcctgggtgacagagtg

SEQ ID NO: 2585 - RNA, 20 nt, synthetic construct
  source 1..20: mol_type = other RNA
gcctgggtgacagagtgagg

SEQ ID NO: 2586 - RNA, 20 nt, synthetic construct
  source 1..20: mol_type = other RNA
tccgcctcactctgtcaccc

SEQ ID NO: 2587 - RNA, 20 nt, synthetic construct
  source 1..20: mol_type = other RNA
aaacaaaaattagccaagcc

SEQ ID NO: 2588 - RNA, 20 nt, synthetic construct
  source 1..20: mol_type = other RNA
caggcgctcgtcaccaggct

SEQ ID NO: 2589 - RNA, 20 nt, synthetic construct
  source 1..20: mol_type = other RNA
gattacaggcgctcgtcacc

SEQ ID NO: 2590 - RNA, 20 nt, synthetic construct
  source 1..20: mol_type = other RNA
gcctgtaatcccagctactc

SEQ ID NO: 2591 - RNA, 20 nt, synthetic construct
  source 1..20: mol_type = other RNA
tgtaatcccagctactcagg

SEQ ID NO: 2592 - RNA, 20 nt, synthetic construct
  source 1..20: mol_type = other RNA
tcctgagtagctgggattac

SEQ ID NO: 2593 - RNA, 20 nt, synthetic construct
  source 1..20: mol_type = other RNA
cccagctactcaggaggctg

SEQ ID NO: 2594 - RNA, 20 nt, synthetic construct
  source 1..20: mol_type = other RNA
cctcagcctcctgagtagct

SEQ ID NO: 2595 - RNA, 20 nt, synthetic construct
  source 1..20: mol_type = other RNA
gcctcagcctcctgagtagc

SEQ ID NO: 2596 - RNA, 20 nt, synthetic construct
  source 1..20: mol_type = other RNA
catgagaatcgcttaaaccc

SEQ ID NO: 2597 - RNA, 20 nt, synthetic construct
  source 1..20: mol_type = other RNA
gagaatcgcttaaacccagg

SEQ ID NO: 2598 - RNA, 20 nt, synthetic construct
  source 1..20: mol_type = other RNA
aatcgcttaaacccaggagg

SEQ ID NO: 2599 - RNA, 20 nt, synthetic construct
  source 1..20: mol_type = other RNA
cgcttaaacccaggaggcgg

SEQ ID NO: 2600 - RNA, 20 nt, synthetic construct
  source 1..20: mol_type = other RNA
cactgcagcctccgcctcct

SEQ ID NO: 2601 - RNA, 20 nt, synthetic construct
  source 1..20: mol_type = other RNA
tcactgcagcctccgcctcc

SEQ ID NO: 2602 - RNA, 20 nt, synthetic construct
  source 1..20: mol_type = other RNA
gcgccactgcaacaaccagc

SEQ ID NO: 2603 - RNA, 20 nt, synthetic construct
  source 1..20: mol_type = other RNA
tgcaacaaccagcaggcctg

SEQ ID NO: 2604 - RNA, 20 nt, synthetic construct
  source 1..20: mol_type = other RNA
aggcctgctggttgttgcag

SEQ ID NO: 2605 - RNA, 20 nt, synthetic construct
  source 1..20: mol_type = other RNA
gcaggcctgaggctcatcct

SEQ ID NO: 2606 - RNA, 20 nt, synthetic construct
  source 1..20: mol_type = other RNA
gggacaaatagttttcagct

SEQ ID NO: 2607 - RNA, 20 nt, synthetic construct
  source 1..20: mol_type = other RNA
tgggacaaatagttttcagc

SEQ ID NO: 2608 - RNA, 20 nt, synthetic construct
  source 1..20: mol_type = other RNA
actatttgtcccagcctcta

SEQ ID NO: 2609 - RNA, 20 nt, synthetic construct
  source 1..20: mol_type = other RNA
gtcacaggaccttagaggct

SEQ ID NO: 2610 - RNA, 20 nt, synthetic construct
  source 1..20: mol_type = other RNA
tgtcacaggaccttagaggc

SEQ ID NO: 2611 - RNA, 20 nt, synthetic construct
  source 1..20: mol_type = other RNA
tctaaggtcctgtgacagtc

SEQ ID NO: 2612 - RNA, 20 nt, synthetic construct
  source 1..20: mol_type = other RNA
agactgtcacaggaccttag

SEQ ID NO: 2613 - RNA, 20 nt, synthetic construct
  source 1..20: mol_type = other RNA
tcctgtgacagtctggccaa

SEQ ID NO: 2614 - RNA, 20 nt, synthetic construct
  source 1..20: mol_type = other RNA
cctgtgacagtctggccaat

SEQ ID NO: 2615 - RNA, 20 nt, synthetic construct
  source 1..20: mol_type = other RNA
cccattggccagactgtcac

SEQ ID NO: 2616 - RNA, 20 nt, synthetic construct
  source 1..20: mol_type = other RNA
tgggaataagcagaaaccac

SEQ ID NO: 2617 - RNA, 20 nt, synthetic construct
  source 1..20: mol_type = other RNA
gggaataagcagaaaccact

SEQ ID NO: 2618 - RNA, 20 nt, synthetic construct
  source 1..20: mol_type = other RNA
ataagcagaaaccactgggt

SEQ ID NO: 2619 - RNA, 20 nt, synthetic construct
  source 1..20: mol_type = other RNA
taagcagaaaccactgggtt

SEQ ID NO: 2620 - RNA, 20 nt, synthetic construct
  source 1..20: mol_type = other RNA
aagcagaaaccactgggttg

SEQ ID NO: 2621 - RNA, 20 nt, synthetic construct
  source 1..20: mol_type = other RNA
aaccactgggttggggctgc

SEQ ID NO: 2622 - RNA, 20 nt, synthetic construct
  source 1..20: mol_type = other RNA
ttcctgcagccccaacccag

SEQ ID NO: 2623 - RNA, 20 nt, synthetic construct
  source 1..20: mol_type = other RNA
gcaggaaaacgctgacaaag

SEQ ID NO: 2624 - RNA, 20 nt, synthetic construct
  source 1..20: mol_type = other RNA
aaaacgctgacaaagaggac

SEQ ID NO: 2625 - RNA, 20 nt, synthetic construct
  source 1..20: mol_type = other RNA
tgacaaagaggactggctcc

SEQ ID NO: 2626 - RNA, 20 nt, synthetic construct
  source 1..20: mol_type = other RNA
gcagtgaggacaaaggtacc

SEQ ID NO: 2627 - RNA, 20 nt, synthetic construct
  source 1..20: mol_type = other RNA
tgtcctcactgctgcctgcc

SEQ ID NO: 2628 - RNA, 20 nt, synthetic construct
  source 1..20: mol_type = other RNA
gcaggcagcagtgaggacaa

SEQ ID NO: 2629 - RNA, 20 nt, synthetic construct
  source 1..20: mol_type = other RNA
gttccaggcaggcagcagtg

SEQ ID NO: 2630 - RNA, 20 nt, synthetic construct
  source 1..20: mol_type = other RNA
gcaaaacctatgttccaggc

SEQ ID NO: 2631 - RNA, 20 nt, synthetic construct
  source 1..20: mol_type = other RNA
tggaacataggttttgctgc

SEQ ID NO: 2632 - RNA, 20 nt, synthetic construct
  source 1..20: mol_type = other RNA
ggaacataggttttgctgcc

SEQ ID NO: 2633 - RNA, 20 nt, synthetic construct
  source 1..20: mol_type = other RNA
gaacataggttttgctgccg

SEQ ID NO: 2634 - RNA, 20 nt, synthetic construct
  source 1..20: mol_type = other RNA
aacataggttttgctgccgg

SEQ ID NO: 2635 - RNA, 20 nt, synthetic construct
  source 1..20: mol_type = other RNA
aggttttgctgccgggggtg

SEQ ID NO: 2636 - RNA, 20 nt, synthetic construct
  source 1..20: mol_type = other RNA
ggttttgctgccgggggtga

SEQ ID NO: 2637 - RNA, 20 nt, synthetic construct
  source 1..20: mol_type = other RNA
gttttgctgccgggggtgag

SEQ ID NO: 2638 - RNA, 20 nt, synthetic construct
  source 1..20: mol_type = other RNA
ttgctgccgggggtgagggg

SEQ ID NO: 2639 - RNA, 20 nt, synthetic construct
  source 1..20: mol_type = other RNA
tgctgccgggggtgaggggt

SEQ ID NO: 2640 - RNA, 20 nt, synthetic construct
  source 1..20: mol_type = other RNA
cgggggtgaggggtgggaac

SEQ ID NO: 2641 - RNA, 20 nt, synthetic construct
  source 1..20: mol_type = other RNA
ctgttcccacccctcacccc

SEQ ID NO: 2642 - RNA, 20 nt, synthetic construct
  source 1..20: mol_type = other RNA
ggagccatcctgtgacagca

SEQ ID NO: 2643 - RNA, 20 nt, synthetic construct
  source 1..20: mol_type = other RNA
tttaccttgctgtcacagga

SEQ ID NO: 2644 - RNA, 20 nt, synthetic construct
  source 1..20: mol_type = other RNA
gcattttaccttgctgtcac

SEQ ID NO: 2645 - RNA, 20 nt, synthetic construct
  source 1..20: mol_type = other RNA
aaaatgcacattcctaagaa

SEQ ID NO: 2646 - RNA, 20 nt, synthetic construct
  source 1..20: mol_type = other RNA
tatttctgcttacctttctt

SEQ ID NO: 2647 - RNA, 20 nt, synthetic construct
  source 1..20: mol_type = other RNA
gaaataccagcattgagtca

SEQ ID NO: 2648 - RNA, 20 nt, synthetic construct
  source 1..20: mol_type = other RNA
aaataccagcattgagtcat

SEQ ID NO: 2649 - RNA, 20 nt, synthetic construct
  source 1..20: mol_type = other RNA
tgtcacccatgactcaatgc

SEQ ID NO: 2650 - RNA, 20 nt, synthetic construct
  source 1..20: mol_type = other RNA
agacttaagggctgttactg

SEQ ID NO: 2651 - RNA, 20 nt, synthetic construct
  source 1..20: mol_type = other RNA
aattctggagagagacttaa

SEQ ID NO: 2652 - RNA, 20 nt, synthetic construct
  source 1..20: mol_type = other RNA
gaattctggagagagactta

SEQ ID NO: 2653 - RNA, 20 nt, synthetic construct
  source 1..20: mol_type = other RNA
ttctcatgtgatatgaattc

SEQ ID NO: 2654 - RNA, 20 nt, synthetic construct
  source 1..20: mol_type = other RNA
acatgagaaacataaactcc

SEQ ID NO: 2655 - RNA, 20 nt, synthetic construct
  source 1..20: mol_type = other RNA
ttcactaggtctatcacata

SEQ ID NO: 2656 - RNA, 20 nt, synthetic construct
  source 1..20: mol_type = other RNA
agccagctctacttgtgttc

SEQ ID NO: 2657 - RNA, 20 nt, synthetic construct
  source 1..20: mol_type = other RNA
ctccagaacacaagtagagc

SEQ ID NO: 2658 - RNA, 20 nt, synthetic construct
  source 1..20: mol_type = other RNA
gaatctgtgatagaagggga

SEQ ID NO: 2659 - RNA, 20 nt, synthetic construct
  source 1..20: mol_type = other RNA
ttcggaatctgtgatagaag

SEQ ID NO: 2660 - RNA, 20 nt, synthetic construct
  source 1..20: mol_type = other RNA
attcggaatctgtgatagaa

SEQ ID NO: 2661 - RNA, 20 nt, synthetic construct
  source 1..20: mol_type = other RNA
cattcggaatctgtgataga

SEQ ID NO: 2662 - RNA, 20 nt, synthetic construct
  source 1..20: mol_type = other RNA
cagattccgaatgtttcctc

SEQ ID NO: 2663 - RNA, 20 nt, synthetic construct
  source 1..20: mol_type = other RNA
agattccgaatgtttcctct

SEQ ID NO: 2664 - RNA, 20 nt, synthetic construct
  source 1..20: mol_type = other RNA
aatgtttcctctgggcacag

SEQ ID NO: 2665 - RNA, 20 nt, synthetic construct
  source 1..20: mol_type = other RNA
ctgtgcccagaggaaacatt

SEQ ID NO: 2666 - RNA, 20 nt, synthetic construct
  source 1..20: mol_type = other RNA
gtgtgagccactgtgcccag

SEQ ID NO: 2667 - RNA, 20 nt, synthetic construct
  source 1..20: mol_type = other RNA
gtggctcacacctgcaatcc

SEQ ID NO: 2668 - RNA, 20 nt, synthetic construct
  source 1..20: mol_type = other RNA
cacctgcaatcctggtgctt

SEQ ID NO: 2669 - RNA, 20 nt, synthetic construct
  source 1..20: mol_type = other RNA
acctgcaatcctggtgcttt

SEQ ID NO: 2670 - RNA, 20 nt, synthetic construct
  source 1..20: mol_type = other RNA
tgcaatcctggtgctttggg

SEQ ID NO: 2671 - RNA, 20 nt, synthetic construct
  source 1..20: mol_type = other RNA
tcccaaagcaccaggattgc

SEQ ID NO: 2672 - RNA, 20 nt, synthetic construct
  source 1..20: mol_type = other RNA
ggtgctttgggaggcccagc

SEQ ID NO: 2673 - RNA, 20 nt, synthetic construct
  source 1..20: mol_type = other RNA
gctgggcctcccaaagcacc

SEQ ID NO: 2674 - RNA, 20 nt, synthetic construct
  source 1..20: mol_type = other RNA
ctttgggaggcccagctgga

SEQ ID NO: 2675 - RNA, 20 nt, synthetic construct
  source 1..20: mol_type = other RNA
ccagctggaaggatcacttg

SEQ ID NO: 2676 - RNA, 20 nt, synthetic construct
  source 1..20: mol_type = other RNA
cagctggaaggatcacttga

SEQ ID NO: 2677 - RNA, 20 nt, synthetic construct
  source 1..20: mol_type = other RNA
ctcaagtgatccttccagct

SEQ ID NO: 2678 - RNA, 20 nt, synthetic construct
  source 1..20: mol_type = other RNA
tggaaggatcacttgagggt

SEQ ID NO: 2679 - RNA, 20 nt, synthetic construct
  source 1..20: mol_type = other RNA
gtaggagtttgagaccagcc

SEQ ID NO: 2680 - RNA, 20 nt, synthetic construct
  source 1..20: mol_type = other RNA
taggagtttgagaccagcct

SEQ ID NO: 2681 - RNA, 20 nt, synthetic construct
  source 1..20: mol_type = other RNA
tcttactgtgttgcccaggc

SEQ ID NO: 2682 - RNA, 20 nt, synthetic construct
  source 1..20: mol_type = other RNA
ggtgtcttactgtgttgccc

SEQ ID NO: 2683 - RNA, 20 nt, synthetic construct
  source 1..20: mol_type = other RNA
aaaaaattttttggcagagc

SEQ ID NO: 2684 - RNA, 20 nt, synthetic construct
  source 1..20: mol_type = other RNA
aaaaaatttttttaattagc

SEQ ID NO: 2685 - RNA, 20 nt, synthetic construct
  source 1..20: mol_type = other RNA
aaaaatttttttaattagct

SEQ ID NO: 2686 - RNA, 20 nt, synthetic construct
  source 1..20: mol_type = other RNA
aaaatttttttaattagctg

SEQ ID NO: 2687 - RNA, 20 nt, synthetic construct
  source 1..20: mol_type = other RNA
agctaattaaaaaaattttt

SEQ ID NO: 2688 - RNA, 20 nt, synthetic construct
  source 1..20: mol_type = other RNA
tttttttaattagctgggga

SEQ ID NO: 2689 - RNA, 20 nt, synthetic construct
  source 1..20: mol_type = other RNA
ttttaattagctggggatgg

SEQ ID NO: 2690 - RNA, 20 nt, synthetic construct
  source 1..20: mol_type = other RNA
catgtgtagttccagcttct

SEQ ID NO: 2691 - RNA, 20 nt, synthetic construct
  source 1..20: mol_type = other RNA
atgtgtagttccagcttctt

SEQ ID NO: 2692 - RNA, 20 nt, synthetic construct
  source 1..20: mol_type = other RNA
tgtagttccagcttcttggg

SEQ ID NO: 2693 - RNA, 20 nt, synthetic construct
  source 1..20: mol_type = other RNA
gcttcttgggaggcagagac

SEQ ID NO: 2694 - RNA, 20 nt, synthetic construct
  source 1..20: mol_type = other RNA
gtctctgcctcccaagaagc

SEQ ID NO: 2695 - RNA, 20 nt, synthetic construct
  source 1..20: mol_type = other RNA
tcttgggaggcagagacagg

SEQ ID NO: 2696 - RNA, 20 nt, synthetic construct
  source 1..20: mol_type = other RNA
caggaggattgcttgaactc

SEQ ID NO: 2697 - RNA, 20 nt, synthetic construct
  source 1..20: mol_type = other RNA
cctgctactgcactctagcc

SEQ ID NO: 2698 - RNA, 20 nt, synthetic construct
  source 1..20: mol_type = other RNA
ctgctactgcactctagcct

SEQ ID NO: 2699 - RNA, 20 nt, synthetic construct
  source 1..20: mol_type = other RNA
ccaggctagagtgcagtagc

SEQ ID NO: 2700 - RNA, 20 nt, synthetic construct
  source 1..20: mol_type = other RNA
ctagcctgggcaacagagta

SEQ ID NO: 2701 - RNA, 20 nt, synthetic construct
  source 1..20: mol_type = other RNA
agggccttactctgttgccc

SEQ ID NO: 2702 - RNA, 20 nt, synthetic construct
  source 1..20: mol_type = other RNA
aaacttttttttttttaaca

SEQ ID NO: 2703 - RNA, 20 nt, synthetic construct
  source 1..20: mol_type = other RNA
gaaacttttttttttttaac

SEQ ID NO: 2704 - RNA, 20 nt, synthetic construct
  source 1..20: mol_type = other RNA
taacaggtttcactgctgat

SEQ ID NO: 2705 - RNA, 20 nt, synthetic construct
  source 1..20: mol_type = other RNA
ttaacaggtttcactgctga

SEQ ID NO: 2706 - RNA, 20 nt, synthetic construct
  source 1..20: mol_type = other RNA
cagtgaaacctgttaatcca

SEQ ID NO: 2707 - RNA, 20 nt, synthetic construct
  source 1..20: mol_type = other RNA
ctgagaaaccttggattaac

SEQ ID NO: 2708 - RNA, 20 nt, synthetic construct
  source 1..20: mol_type = other RNA
gtgctgaggctgagaaacct

SEQ ID NO: 2709 - RNA, 20 nt, synthetic construct
  source 1..20: mol_type = other RNA
ctcagcactactgacatttt

SEQ ID NO: 2710 - RNA, 20 nt, synthetic construct
  source 1..20: mol_type = other RNA
ctaaaatgtcagtagtgctg

SEQ ID NO: 2711 - RNA, 20 nt, synthetic construct
  source 1..20: mol_type = other RNA
ttaggctagctaattttttt

SEQ ID NO: 2712 - RNA, 20 nt, synthetic construct
  source 1..20: mol_type = other RNA
taggctagctaatttttttt

SEQ ID NO: 2713 - RNA, 20 nt, synthetic construct
  source 1..20: mol_type = other RNA
aggctagctaattttttttg

SEQ ID NO: 2714 - RNA, 20 nt, synthetic construct
  source 1..20: mol_type = other RNA
ggctagctaattttttttgg

SEQ ID NO: 2715 - RNA, 20 nt, synthetic construct
  source 1..20: mol_type = other RNA
gctagctaattttttttggg

SEQ ID NO: 2716 - RNA, 20 nt, synthetic construct
  source 1..20: mol_type = other RNA
ctagctaattttttttgggg

SEQ ID NO: 2717 - RNA, 20 nt, synthetic construct
  source 1..20: mol_type = other RNA
tagctaattttttttggggg

SEQ ID NO: 2718 - RNA, 20 nt, synthetic construct
  source 1..20: mol_type = other RNA
agctaattttttttgggggg

SEQ ID NO: 2719 - RNA, 20 nt, synthetic construct
  source 1..20: mol_type = other RNA
gctaattttttttggggggg

SEQ ID NO: 2720 - RNA, 20 nt, synthetic construct
  source 1..20: mol_type = other RNA
ctaattttttttgggggggg

SEQ ID NO: 2721 - RNA, 20 nt, synthetic construct
  source 1..20: mol_type = other RNA
taattttttttggggggggg

SEQ ID NO: 2722 - RNA, 20 nt, synthetic construct
  source 1..20: mol_type = other RNA
aattttttttgggggggggg

SEQ ID NO: 2723 - RNA, 20 nt, synthetic construct
  source 1..20: mol_type = other RNA
tttgggggggggggggcaag

SEQ ID NO: 2724 - RNA, 20 nt, synthetic construct
  source 1..20: mol_type = other RNA
ttgggggggggggggcaagt

SEQ ID NO: 2725 - RNA, 20 nt, synthetic construct
  source 1..20: mol_type = other RNA
tgggggggggggggcaagtg

SEQ ID NO: 2726 - RNA, 20 nt, synthetic construct
  source 1..20: mol_type = other RNA
gggactgtcttgtgtattgc

SEQ ID NO: 2727 - RNA, 20 nt, synthetic construct
  source 1..20: mol_type = other RNA
atgtttagcagcagcatccc

SEQ ID NO: 2728 - RNA, 20 nt, synthetic construct
  source 1..20: mol_type = other RNA
catctaatgggtagaggcca

SEQ ID NO: 2729 - RNA, 20 nt, synthetic construct
  source 1..20: mol_type = other RNA
acatctaatgggtagaggcc

SEQ ID NO: 2730 - RNA, 20 nt, synthetic construct
  source 1..20: mol_type = other RNA
ctctacccattagatgtcag

SEQ ID NO: 2731 - RNA, 20 nt, synthetic construct
  source 1..20: mol_type = other RNA
cactgacatctaatgggtag

SEQ ID NO: 2732 - RNA, 20 nt, synthetic construct
  source 1..20: mol_type = other RNA
gggtgccactgacatctaat

SEQ ID NO: 2733 - RNA, 20 nt, synthetic construct
  source 1..20: mol_type = other RNA
ggggtgccactgacatctaa

SEQ ID NO: 2734 - RNA, 20 nt, synthetic construct
  source 1..20: mol_type = other RNA
gttgttacagatgcagggag

SEQ ID NO: 2735 - RNA, 20 nt, synthetic construct
  source 1..20: mol_type = other RNA
ggttgttacagatgcaggga

SEQ ID NO: 2736 - RNA, 20 nt, synthetic construct
  source 1..20: mol_type = other RNA
tggttgttacagatgcaggg

SEQ ID NO: 2737 - RNA, 20 nt, synthetic construct
  source 1..20: mol_type = other RNA
ttttggttgttacagatgca

SEQ ID NO: 2738 - RNA, 20 nt, synthetic construct
  source 1..20: mol_type = other RNA
gttttggttgttacagatgc

SEQ ID NO: 2739 - RNA, 20 nt, synthetic construct
  source 1..20: mol_type = other RNA
taacaaccaaaactctctcc

SEQ ID NO: 2740 - RNA, 20 nt, synthetic construct
  source 1..20: mol_type = other RNA
gcaatgcctggagagagttt

SEQ ID NO: 2741 - RNA, 20 nt, synthetic construct
  source 1..20: mol_type = other RNA
gaaggacatttggcaatgcc

SEQ ID NO: 2742 - RNA, 20 nt, synthetic construct
  source 1..20: mol_type = other RNA
ttttgctgtggaaggacatt

SEQ ID NO: 2743 - RNA, 20 nt, synthetic construct
  source 1..20: mol_type = other RNA
atgatggattttgctgtgga

SEQ ID NO: 2744 - RNA, 20 nt, synthetic construct
  source 1..20: mol_type = other RNA
gttcatgatggattttgctg

SEQ ID NO: 2745 - RNA, 20 nt, synthetic construct
  source 1..20: mol_type = other RNA
ggtgggggatatgttcatga

SEQ ID NO: 2746 - RNA, 20 nt, synthetic construct
  source 1..20: mol_type = other RNA
gttctctactgtgttggtgg

SEQ ID NO: 2747 - RNA, 20 nt, synthetic construct
  source 1..20: mol_type = other RNA
ggttctctactgtgttggtg

SEQ ID NO: 2748 - RNA, 20 nt, synthetic construct
  source 1..20: mol_type = other RNA
tggttctctactgtgttggt

SEQ ID NO: 2749 - RNA, 20 nt, synthetic construct
  source 1..20: mol_type = other RNA
gtggttctctactgtgttgg

SEQ ID NO: 2750 - RNA, 20 nt, synthetic construct
  source 1..20: mol_type = other RNA
acggtggttctctactgtgt

SEQ ID NO: 2751 - RNA, 20 nt, synthetic construct
  source 1..20: mol_type = other RNA
ttggtattaaatgagaacgg

SEQ ID NO: 2752 - RNA, 20 nt, synthetic construct
  source 1..20: mol_type = other RNA
agtttggtattaaatgagaa

SEQ ID NO: 2753 - RNA, 20 nt, synthetic construct
  source 1..20: mol_type = other RNA
aataccaaactagatctaaa

SEQ ID NO: 2754 - RNA, 20 nt, synthetic construct
  source 1..20: mol_type = other RNA
caaactagatctaaatggca

SEQ ID NO: 2755 - RNA, 20 nt, synthetic construct
  source 1..20: mol_type = other RNA
cttgccatttagatctagtt

SEQ ID NO: 2756 - RNA, 20 nt, synthetic construct
  source 1..20: mol_type = other RNA
ataattagatttaaaatttt

SEQ ID NO: 2757 - RNA, 20 nt, synthetic construct
  source 1..20: mol_type = other RNA
atttttgctcaaaaaaagca

SEQ ID NO: 2758 - RNA, 20 nt, synthetic construct
  source 1..20: mol_type = other RNA
ctagttaatttctttcttag

SEQ ID NO: 2759 - RNA, 20 nt, synthetic construct
  source 1..20: mol_type = other RNA
gtggcaatgatccaaaatgt

SEQ ID NO: 2760 - RNA, 20 nt, synthetic construct
  source 1..20: mol_type = other RNA
gctatgagttgcctacattt

SEQ ID NO: 2761 - RNA, 20 nt, synthetic construct
  source 1..20: mol_type = other RNA
cagttacttataatgttgaa

SEQ ID NO: 2762 - RNA, 20 nt, synthetic construct
  source 1..20: mol_type = other RNA
tctaatgacaaagaaaagac

SEQ ID NO: 2763 - RNA, 20 nt, synthetic construct
  source 1..20: mol_type = other RNA
aagactggttgaataaatcg

SEQ ID NO: 2764 - RNA, 20 nt, synthetic construct
  source 1..20: mol_type = other RNA
agagctgcatgatattcact

SEQ ID NO: 2765 - RNA, 20 nt, synthetic construct
  source 1..20: mol_type = other RNA
catgcagctcttttaaaaac

SEQ ID NO: 2766 - RNA, 20 nt, synthetic construct
  source 1..20: mol_type = other RNA
aacaggccctcataccaaat

SEQ ID NO: 2767 - RNA, 20 nt, synthetic construct
  source 1..20: mol_type = other RNA
ctactgccaatttggtatga

SEQ ID NO: 2768 - RNA, 20 nt, synthetic construct
  source 1..20: mol_type = other RNA
gctactgccaatttggtatg

SEQ ID NO: 2769 - RNA, 20 nt, synthetic construct
  source 1..20: mol_type = other RNA
agtttatgctactgccaatt

SEQ ID NO: 2770 - RNA, 20 nt, synthetic construct
  source 1..20: mol_type = other RNA
agcataaactcacaatctct

SEQ ID NO: 2771 - RNA, 20 nt, synthetic construct
  source 1..20: mol_type = other RNA
ataatatatgacataaacaa

SEQ ID NO: 2772 - RNA, 20 nt, synthetic construct
  source 1..20: mol_type = other RNA
aggaaaaacaaatcagtaaa

SEQ ID NO: 2773 - RNA, 20 nt, synthetic construct
  source 1..20: mol_type = other RNA
tattattaatacacgctatt

SEQ ID NO: 2774 - RNA, 20 nt, synthetic construct
  source 1..20: mol_type = other RNA
aatacagctaaggagctaag

SEQ ID NO: 2775 - RNA, 20 nt, synthetic construct
  source 1..20: mol_type = other RNA
ttaagtttcaaatacagcta

SEQ ID NO: 2776 - RNA, 20 nt, synthetic construct
  source 1..20: mol_type = other RNA
gtggtgtgtggtcttaatgt

SEQ ID NO: 2777 - RNA, 20 nt, synthetic construct
  source 1..20: mol_type = other RNA
ctttggaaaaaggtggtgtg

SEQ ID NO: 2778 - RNA, 20 nt, synthetic construct
  source 1..20: mol_type = other RNA
tagactactttggaaaaagg

SEQ ID NO: 2779 - RNA, 20 nt, synthetic construct
  source 1..20: mol_type = other RNA
ttccaaagtagtctaatttt

SEQ ID NO: 2780 - RNA, 20 nt, synthetic construct
  source 1..20: mol_type = other RNA
ttccaaaaattagactactt

SEQ ID NO: 2781 - RNA, 20 nt, synthetic construct
  source 1..20: mol_type = other RNA
atttttggaacattatgaaa

SEQ ID NO: 2782 - RNA, 20 nt, synthetic construct
  source 1..20: mol_type = other RNA
aaatggtccattctgatcaa

SEQ ID NO: 2783 - RNA, 20 nt, synthetic construct
  source 1..20: mol_type = other RNA
tataaggccattgatcagaa

SEQ ID NO: 2784 - RNA, 20 nt, synthetic construct
  source 1..20: mol_type = other RNA
gggcatggagataagctata

SEQ ID NO: 2785 - RNA, 20 nt, synthetic construct
  source 1..20: mol_type = other RNA
caatttaaaatctttgggca

SEQ ID NO: 2786 - RNA, 20 nt, synthetic construct
  source 1..20: mol_type = other RNA
gtttacaatttaaaatcttt

SEQ ID NO: 2787 - RNA, 20 nt, synthetic construct
  source 1..20: mol_type = other RNA
tgtttacaatttaaaatctt

SEQ ID NO: 2788 - RNA, 20 nt, synthetic construct
  source 1..20: mol_type = other RNA
caaaaaaaaaaaaggaaagt

SEQ ID NO: 2789 - RNA, 20 nt, synthetic construct
  source 1..20: mol_type = other RNA
ctctgtctcaaaaaaaaaaa

SEQ ID NO: 2790 - RNA, 20 nt, synthetic construct
  source 1..20: mol_type = other RNA
cagagtcttgctctgttgcc

SEQ ID NO: 2791 - RNA, 20 nt, synthetic construct
  source 1..20: mol_type = other RNA
tcttgctctgttgccaggct

SEQ ID NO: 2792 - RNA, 20 nt, synthetic construct
  source 1..20: mol_type = other RNA
cttgctctgttgccaggcta

SEQ ID NO: 2793 - RNA, 20 nt, synthetic construct
  source 1..20: mol_type = other RNA
gttgccaggctagggtgcag

SEQ ID NO: 2794 - RNA, 20 nt, synthetic construct
  source 1..20: mol_type = other RNA
tgcaccactgcaccctagcc

SEQ ID NO: 2795 - RNA, 20 nt, synthetic construct
  source 1..20: mol_type = other RNA
agggtgcagtggtgcaatct

SEQ ID NO: 2796 - RNA, 20 nt, synthetic construct
  source 1..20: mol_type = other RNA
tcactgcaacctcagcctcc

SEQ ID NO: 2797 - RNA, 20 nt, synthetic construct
  source 1..20: mol_type = other RNA
cactgcaacctcagcctcca

SEQ ID NO: 2798 - RNA, 20 nt, synthetic construct
  source 1..20: mol_type = other RNA
cgatttaaccctggaggctg

SEQ ID NO: 2799 - RNA, 20 nt, synthetic construct
  source 1..20: mol_type = other RNA
gagaatcgatttaaccctgg

SEQ ID NO: 2800 - RNA, 20 nt, synthetic construct
  source 1..20: mol_type = other RNA
caggagaatcgatttaaccc

SEQ ID NO: 2801 - RNA, 20 nt, synthetic construct
  source 1..20: mol_type = other RNA
gcctcagcctcccgagtagc

SEQ ID NO: 2802 - RNA, 20 nt, synthetic construct
  source 1..20: mol_type = other RNA
cctcagcctcccgagtagct

SEQ ID NO: 2803 - RNA, 20 nt, synthetic construct
  source 1..20: mol_type = other RNA
gctactcgggaggctgaggc

SEQ ID NO: 2804 - RNA, 20 nt, synthetic construct
  source 1..20: mol_type = other RNA
cccagctactcgggaggctg

SEQ ID NO: 2805 - RNA, 20 nt, synthetic construct
  source 1..20: mol_type = other RNA
tgtggtcccagctactcggg

SEQ ID NO: 2806 - RNA, 20 nt, synthetic construct
  source 1..20: mol_type = other RNA
atttgtggtcccagctactc

SEQ ID NO: 2807 - RNA, 20 nt, synthetic construct
  source 1..20: mol_type = other RNA
catttgtggtcccagctact

SEQ ID NO: 2808 - RNA, 20 nt, synthetic construct
  source 1..20: mol_type = other RNA
caaatgcccgccaccacgcc

SEQ ID NO: 2809 - RNA, 20 nt, synthetic construct
  source 1..20: mol_type = other RNA
ggcgtggtggcgggcatttg

SEQ ID NO: 2810 - RNA, 20 nt, synthetic construct
  source 1..20: mol_type = other RNA
aattagccgggcgtggtggc

SEQ ID NO: 2811 - RNA, 20 nt, synthetic construct
  source 1..20: mol_type = other RNA
aaattagccgggcgtggtgg

SEQ ID NO: 2812 - RNA, 20 nt, synthetic construct
  source 1..20: mol_type = other RNA
aaaaaattagccgggcgtgg

SEQ ID NO: 2813 - RNA, 20 nt, synthetic construct
  source 1..20: mol_type = other RNA
aaaaaaaaattagccgggcg

SEQ ID NO: 2814 - RNA, 20 nt, synthetic construct
  source 1..20: mol_type = other RNA
aatacaaaaaaaaattagcc

SEQ ID NO: 2815 - RNA, 20 nt, synthetic construct
  source 1..20: mol_type = other RNA
aaatacaaaaaaaaattagc

SEQ ID NO: 2816 - RNA, 20 nt, synthetic construct
  source 1..20: mol_type = other RNA
ttttgtatttttagtagaga

SEQ ID NO: 2817 - RNA, 20 nt, synthetic construct
  source 1..20: mol_type = other RNA
tttgtatttttagtagagac

SEQ ID NO: 2818 - RNA, 20 nt, synthetic construct
  source 1..20: mol_type = other RNA
ttgtatttttagtagagacg

SEQ ID NO: 2819 - RNA, 20 nt, synthetic construct
  source 1..20: mol_type = other RNA
ggggtttcaccgtgttagcc

SEQ ID NO: 2820 - RNA, 20 nt, synthetic construct
  source 1..20: mol_type = other RNA
tttcaccgtgttagccagga

SEQ ID NO: 2821 - RNA, 20 nt, synthetic construct
  source 1..20: mol_type = other RNA
cgagaccatcctggctaaca

SEQ ID NO: 2822 - RNA, 20 nt, synthetic construct
  source 1..20: mol_type = other RNA
tcaggagatcgagaccatcc

SEQ ID NO: 2823 - RNA, 20 nt, synthetic construct
  source 1..20: mol_type = other RNA
ggcgggcagatcacgaggtc

SEQ ID NO: 2824 - RNA, 20 nt, synthetic construct
  source 1..20: mol_type = other RNA
gctgaggcgggcagatcacg

SEQ ID NO: 2825 - RNA, 20 nt, synthetic construct
  source 1..20: mol_type = other RNA
gcctcagcctcccaaagtgc

SEQ ID NO: 2826 - RNA, 20 nt, synthetic construct
  source 1..20: mol_type = other RNA
cctcagcctcccaaagtgct

SEQ ID NO: 2827 - RNA, 20 nt, synthetic construct
  source 1..20: mol_type = other RNA
gcactttgggaggctgaggc

SEQ ID NO: 2828 - RNA, 20 nt, synthetic construct
  source 1..20: mol_type = other RNA
agcactttgggaggctgagg

SEQ ID NO: 2829 - RNA, 20 nt, synthetic construct
  source 1..20: mol_type = other RNA
cccagcactttgggaggctg

SEQ ID NO: 2830 - RNA, 20 nt, synthetic construct
  source 1..20: mol_type = other RNA
tcccaaagtgctgggattac

SEQ ID NO: 2831 - RNA, 20 nt, synthetic construct
  source 1..20: mol_type = other RNA
tgtaatcccagcactttggg

SEQ ID NO: 2832 - RNA, 20 nt, synthetic construct
  source 1..20: mol_type = other RNA
gcctgtaatcccagcacttt

SEQ ID NO: 2833 - RNA, 20 nt, synthetic construct
  source 1..20: mol_type = other RNA
tgcctgtaatcccagcactt

SEQ ID NO: 2834 - RNA, 20 nt, synthetic construct
  source 1..20: mol_type = other RNA
caggcataagccaccgcgcc

SEQ ID NO: 2835 - RNA, 20 nt, synthetic construct
  source 1..20: mol_type = other RNA
tatgttcaggccaggcgcgg

SEQ ID NO: 2836 - RNA, 20 nt, synthetic construct
  source 1..20: mol_type = other RNA
aggtatgttcaggccaggcg

SEQ ID NO: 2837 - RNA, 20 nt, synthetic construct
  source 1..20: mol_type = other RNA
aaagtaggtatgttcaggcc

SEQ ID NO: 2838 - RNA, 20 nt, synthetic construct
  source 1..20: mol_type = other RNA
cattgaaagtaggtatgttc

SEQ ID NO: 2839 - RNA, 20 nt, synthetic construct
  source 1..20: mol_type = other RNA
aaagtaaacacattgaaagt

SEQ ID NO: 2840 - RNA, 20 nt, synthetic construct
  source 1..20: mol_type = other RNA
atattaggaggtgaaataat

SEQ ID NO: 2841 - RNA, 20 nt, synthetic construct
  source 1..20: mol_type = other RNA
tattatgtgaaaatattagg

SEQ ID NO: 2842 - RNA, 20 nt, synthetic construct
  source 1..20: mol_type = other RNA
tgttattatgtgaaaatatt

SEQ ID NO: 2843 - RNA, 20 nt, synthetic construct
  source 1..20: mol_type = other RNA
tctcaaagcaaatttcaaga

SEQ ID NO: 2844 - RNA, 20 nt, synthetic construct
  source 1..20: mol_type = other RNA
atctcaaagcaaatttcaag

SEQ ID NO: 2845 - RNA, 20 nt, synthetic construct
  source 1..20: mol_type = other RNA
tgctttgagatatatatgca

SEQ ID NO: 2846 - RNA, 20 nt, synthetic construct
  source 1..20: mol_type = other RNA
tatatgcatggcttaaaata

SEQ ID NO: 2847 - RNA, 20 nt, synthetic construct
  source 1..20: mol_type = other RNA
tactatagaaataattttgc

SEQ ID NO: 2848 - RNA, 20 nt, synthetic construct
  source 1..20: mol_type = other RNA
actatagaaataattttgct

SEQ ID NO: 2849 - RNA, 20 nt, synthetic construct
  source 1..20: mol_type = other RNA
ttgctgggttcaaataatgc

SEQ ID NO: 2850 - RNA, 20 nt, synthetic construct
  source 1..20: mol_type = other RNA
tgctgggttcaaataatgct

SEQ ID NO: 2851 - RNA, 20 nt, synthetic construct
  source 1..20: mol_type = other RNA
aagcagtaactgtgcctaaa

SEQ ID NO: 2852 - RNA, 20 nt, synthetic construct
  source 1..20: mol_type = other RNA
aaatggtactgtttaaatac

SEQ ID NO: 2853 - RNA, 20 nt, synthetic construct
  source 1..20: mol_type = other RNA
aatggtactgtttaaataca

SEQ ID NO: 2854 - RNA, 20 nt, synthetic construct
  source 1..20: mol_type = other RNA
gtatttaaacagtaccattt

SEQ ID NO: 2855 - RNA, 20 nt, synthetic construct
  source 1..20: mol_type = other RNA
cagggactctcaaaagtctc

SEQ ID NO: 2856 - RNA, 20 nt, synthetic construct
  source 1..20: mol_type = other RNA
ctttatgtgaagtatacttt

SEQ ID NO: 2857 - RNA, 20 nt, synthetic construct
  source 1..20: mol_type = other RNA
aattctgtgattctcttgaa

SEQ ID NO: 2858 - RNA, 20 nt, synthetic construct
  source 1..20: mol_type = other RNA
agagaatcacagaattcaga

SEQ ID NO: 2859 - RNA, 20 nt, synthetic construct
  source 1..20: mol_type = other RNA
atagaatcctcaaactaact

SEQ ID NO: 2860 - RNA, 20 nt, synthetic construct
  source 1..20: mol_type = other RNA
tcaaactaacttggtgttat

SEQ ID NO: 2861 - RNA, 20 nt, synthetic construct
  source 1..20: mol_type = other RNA
tataacaccaagttagtttg

SEQ ID NO: 2862 - RNA, 20 nt, synthetic construct
  source 1..20: mol_type = other RNA
actaacttggtgttatagga

SEQ ID NO: 2863 - RNA, 20 nt, synthetic construct
  source 1..20: mol_type = other RNA
gatggtcttgaaagaaactg

SEQ ID NO: 2864 - RNA, 20 nt, synthetic construct
  source 1..20: mol_type = other RNA
tcttgaaagaaactgaggcc

SEQ ID NO: 2865 - RNA, 20 nt, synthetic construct
  source 1..20: mol_type = other RNA
caggcatgactcacagcgcc

SEQ ID NO: 2866 - RNA, 20 nt, synthetic construct
  source 1..20: mol_type = other RNA
tgcctgcaatcccaatactt

SEQ ID NO: 2867 - RNA, 20 nt, synthetic construct
  source 1..20: mol_type = other RNA
gcctgcaatcccaatacttt

SEQ ID NO: 2868 - RNA, 20 nt, synthetic construct
  source 1..20: mol_type = other RNA
tgcaatcccaatactttggg

SEQ ID NO: 2869 - RNA, 20 nt, synthetic construct
  source 1..20: mol_type = other RNA
tcccaaagtattgggattgc

SEQ ID NO: 2870 - RNA, 20 nt, synthetic construct
  source 1..20: mol_type = other RNA
cccaatactttgggaggctg

SEQ ID NO: 2871 - RNA, 20 nt, synthetic construct
  source 1..20: mol_type = other RNA
aatactttgggaggctgagg

SEQ ID NO: 2872 - RNA, 20 nt, synthetic construct
  source 1..20: mol_type = other RNA
atactttgggaggctgaggt

SEQ ID NO: 2873 - RNA, 20 nt, synthetic construct
  source 1..20: mol_type = other RNA
cctcagcctcccaaagtatt

SEQ ID NO: 2874 - RNA, 20 nt, synthetic construct
  source 1..20: mol_type = other RNA
acctcagcctcccaaagtat

SEQ ID NO: 2875 - RNA, 20 nt, synthetic construct
  source 1..20: mol_type = other RNA
agaatcacttgagaccagtc

SEQ ID NO: 2876 - RNA, 20 nt, synthetic construct
  source 1..20: mol_type = other RNA
gaatcacttgagaccagtct

SEQ ID NO: 2877 - RNA, 20 nt, synthetic construct
  source 1..20: mol_type = other RNA
tctgtctgtgttgcccagac

SEQ ID NO: 2878 - RNA, 20 nt, synthetic construct
  source 1..20: mol_type = other RNA
aaattttttaatagagatgg

SEQ ID NO: 2879 - RNA, 20 nt, synthetic construct
  source 1..20: mol_type = other RNA
aaaattttttaatagagatg

SEQ ID NO: 2880 - RNA, 20 nt, synthetic construct
  source 1..20: mol_type = other RNA
taaaattttttaatagagat

SEQ ID NO: 2881 - RNA, 20 nt, synthetic construct
  source 1..20: mol_type = other RNA
ttaaaattttttaatagaga

SEQ ID NO: 2882 - RNA, 20 nt, synthetic construct
  source 1..20: mol_type = other RNA
aaaaaattttaaaattagca

SEQ ID NO: 2883 - RNA, 20 nt, synthetic construct
  source 1..20: mol_type = other RNA
attttaaaattagcaaggca

SEQ ID NO: 2884 - RNA, 20 nt, synthetic construct
  source 1..20: mol_type = other RNA
ttaaaattagcaaggcatgg

SEQ ID NO: 2885 - RNA, 20 nt, synthetic construct
  source 1..20: mol_type = other RNA
ggcatggtggtacacatctg

SEQ ID NO: 2886 - RNA, 20 nt, synthetic construct
  source 1..20: mol_type = other RNA
catctgtggtcccagctact

SEQ ID NO: 2887 - RNA, 20 nt, synthetic construct
  source 1..20: mol_type = other RNA
atctgtggtcccagctactt

SEQ ID NO: 2888 - RNA, 20 nt, synthetic construct
  source 1..20: mol_type = other RNA
tgtggtcccagctacttggg

SEQ ID NO: 2889 - RNA, 20 nt, synthetic construct
  source 1..20: mol_type = other RNA
agctacttgggaggcagaag

SEQ ID NO: 2890 - RNA, 20 nt, synthetic construct
  source 1..20: mol_type = other RNA
gctacttgggaggcagaagt

SEQ ID NO: 2891 - RNA, 20 nt, synthetic construct
  source 1..20: mol_type = other RNA
cttctgcctcccaagtagct

SEQ ID NO: 2892 - RNA, 20 nt, synthetic construct
  source 1..20: mol_type = other RNA
acttctgcctcccaagtagc

SEQ ID NO: 2893 - RNA, 20 nt, synthetic construct
  source 1..20: mol_type = other RNA
acttgggaggcagaagtggg

SEQ ID NO: 2894 - RNA, 20 nt, synthetic construct
  source 1..20: mol_type = other RNA
tgggaggatcacttgagctc

SEQ ID NO: 2895 - RNA, 20 nt, synthetic construct
  source 1..20: mol_type = other RNA
gaggatcacttgagctcagg

SEQ ID NO: 2896 - RNA, 20 nt, synthetic construct
  source 1..20: mol_type = other RNA
ggcatgcagtggcgtgatca

SEQ ID NO: 2897 - RNA, 20 nt, synthetic construct
  source 1..20: mol_type = other RNA
cacgccactgcatgccagcc

SEQ ID NO: 2898 - RNA, 20 nt, synthetic construct
  source 1..20: mol_type = other RNA
ttgtccaggctggcatgcag

SEQ ID NO: 2899 - RNA, 20 nt, synthetic construct
  source 1..20: mol_type = other RNA
tcttgctctgttgtccaggc

SEQ ID NO: 2900 - RNA, 20 nt, synthetic construct
  source 1..20: mol_type = other RNA
agagtcttgctctgttgtcc

SEQ ID NO: 2901 - RNA, 20 nt, synthetic construct
  source 1..20: mol_type = other RNA
aaaaaaaaaaaaaaagagag

SEQ ID NO: 2902 - RNA, 20 nt, synthetic construct
  source 1..20: mol_type = other RNA
aaaaaaaaaaaagagagagg

SEQ ID NO: 2903 - RNA, 20 nt, synthetic construct
  source 1..20: mol_type = other RNA
aaaaaaaaaaagagagaggc

SEQ ID NO: 2904 - RNA, 20 nt, synthetic construct
  source 1..20: mol_type = other RNA
aaaaaaaaaagagagaggcg

SEQ ID NO: 2905 - RNA, 20 nt, synthetic construct
  source 1..20: mol_type = other RNA
aagagagaggcggggcacag

SEQ ID NO: 2906 - RNA, 20 nt, synthetic construct
  source 1..20: mol_type = other RNA
tgcctgtaatcctagcactt

SEQ ID NO: 2907 - RNA, 20 nt, synthetic construct
  source 1..20: mol_type = other RNA
tgtaatcctagcactttgga

SEQ ID NO: 2908 - RNA, 20 nt, synthetic construct
  source 1..20: mol_type = other RNA
ttccaaagtgctaggattac

SEQ ID NO: 2909 - RNA, 20 nt, synthetic construct
  source 1..20: mol_type = other RNA
cctagcactttggaaggctg

SEQ ID NO: 2910 - RNA, 20 nt, synthetic construct
  source 1..20: mol_type = other RNA
agcactttggaaggctgagg

SEQ ID NO: 2911 - RNA, 20 nt, synthetic construct
  source 1..20: mol_type = other RNA
gcactttggaaggctgaggt

SEQ ID NO: 2912 - RNA, 20 nt, synthetic construct
  source 1..20: mol_type = other RNA
cctcagccttccaaagtgct

SEQ ID NO: 2913 - RNA, 20 nt, synthetic construct
  source 1..20: mol_type = other RNA
ctttggaaggctgaggtggg

SEQ ID NO: 2914 - RNA, 20 nt, synthetic construct
  source 1..20: mol_type = other RNA
tgaggtgggtggatcgcctg

SEQ ID NO: 2915 - RNA, 20 nt, synthetic construct
  source 1..20: mol_type = other RNA
ggtctcaaactcttgacctc

SEQ ID NO: 2916 - RNA, 20 nt, synthetic construct
  source 1..20: mol_type = other RNA
tcaagagtttgagaccagcc

SEQ ID NO: 2917 - RNA, 20 nt, synthetic construct
  source 1..20: mol_type = other RNA
tgagaccagcctggtcaaca

SEQ ID NO: 2918 - RNA, 20 nt, synthetic construct
  source 1..20: mol_type = other RNA
tttcaccgtgttgaccaggc

SEQ ID NO: 2919 - RNA, 20 nt, synthetic construct
  source 1..20: mol_type = other RNA
agggtttcaccgtgttgacc

SEQ ID NO: 2920 - RNA, 20 nt, synthetic construct
  source 1..20: mol_type = other RNA
aacacggtgaaaccctgctg

SEQ ID NO: 2921 - RNA, 20 nt, synthetic construct
  source 1..20: mol_type = other RNA
acggtgaaaccctgctgagg

SEQ ID NO: 2922 - RNA, 20 nt, synthetic construct
  source 1..20: mol_type = other RNA
cggtgaaaccctgctgaggt

SEQ ID NO: 2923 - RNA, 20 nt, synthetic construct
  source 1..20: mol_type = other RNA
gcaatctgcccacctcagca

SEQ ID NO: 2924 - RNA, 20 nt, synthetic construct
  source 1..20: mol_type = other RNA
ggcaatctgcccacctcagc

SEQ ID NO: 2925 - RNA, 20 nt, synthetic construct
  source 1..20: mol_type = other RNA
tgggcagattgcctgagctc

SEQ ID NO: 2926 - RNA, 20 nt, synthetic construct
  source 1..20: mol_type = other RNA
ggtctcaaactcctgagctc

SEQ ID NO: 2927 - RNA, 20 nt, synthetic construct
  source 1..20: mol_type = other RNA
tcaggagtttgagaccagcc

SEQ ID NO: 2928 - RNA, 20 nt, synthetic construct
  source 1..20: mol_type = other RNA
caggagtttgagaccagcct

SEQ ID NO: 2929 - RNA, 20 nt, synthetic construct
  source 1..20: mol_type = other RNA
tgagaccagcctgggcaaca

SEQ ID NO: 2930 - RNA, 20 nt, synthetic construct
  source 1..20: mol_type = other RNA
tttcaccatgttgcccaggc

SEQ ID NO: 2931 - RNA, 20 nt, synthetic construct
  source 1..20: mol_type = other RNA
agggtttcaccatgttgccc

SEQ ID NO: 2932 - RNA, 20 nt, synthetic construct
  source 1..20: mol_type = other RNA
tttttattttagtagagaca

SEQ ID NO: 2933 - RNA, 20 nt, synthetic construct
  source 1..20: mol_type = other RNA
ctttttattttagtagagac

SEQ ID NO: 2934 - RNA, 20 nt, synthetic construct
  source 1..20: mol_type = other RNA
ctaaaataaaaagagtgagc

SEQ ID NO: 2935 - RNA, 20 nt, synthetic construct
  source 1..20: mol_type = other RNA
taaaataaaaagagtgagct

SEQ ID NO: 2936 - RNA, 20 nt, synthetic construct
  source 1..20: mol_type = other RNA
gctgggcaaaaagagtgagc

SEQ ID NO: 2937 - RNA, 20 nt, synthetic construct
  source 1..20: mol_type = other RNA
ctgggcaaaaagagtgagct

SEQ ID NO: 2938 - RNA, 20 nt, synthetic construct
  source 1..20: mol_type = other RNA
aaagagtgagctgggcgtca

SEQ ID NO: 2939 - RNA, 20 nt, synthetic construct
  source 1..20: mol_type = other RNA
tgtctgtagtcccagctact

SEQ ID NO: 2940 - RNA, 20 nt, synthetic construct
  source 1..20: mol_type = other RNA
tgtagtcccagctactcgga

SEQ ID NO: 2941 - RNA, 20 nt, synthetic construct
  source 1..20: mol_type = other RNA
cccagctactcggaaggctg

SEQ ID NO: 2942 - RNA, 20 nt, synthetic construct
  source 1..20: mol_type = other RNA
cctcagccttccgagtagct

SEQ ID NO: 2943 - RNA, 20 nt, synthetic construct
  source 1..20: mol_type = other RNA
tcctcagccttccgagtagc

SEQ ID NO: 2944 - RNA, 20 nt, synthetic construct
  source 1..20: mol_type = other RNA
aacgagaattgcttgaaccc

SEQ ID NO: 2945 - RNA, 20 nt, synthetic construct
  source 1..20: mol_type = other RNA
gagaattgcttgaacccagg

SEQ ID NO: 2946 - RNA, 20 nt, synthetic construct
  source 1..20: mol_type = other RNA
aattgcttgaacccaggagg

SEQ ID NO: 2947 - RNA, 20 nt, synthetic construct
  source 1..20: mol_type = other RNA
tgcttgaacccaggaggcgg

SEQ ID NO: 2948 - RNA, 20 nt, synthetic construct
  source 1..20: mol_type = other RNA
cactgcaacctccgcctcct

SEQ ID NO: 2949 - RNA, 20 nt, synthetic construct
  source 1..20: mol_type = other RNA
tcactgcaacctccgcctcc

SEQ ID NO: 2950 - RNA, 20 nt, synthetic construct
  source 1..20: mol_type = other RNA
ggagtgcagtggcgttatct

SEQ ID NO: 2951 - RNA, 20 nt, synthetic construct
  source 1..20: mol_type = other RNA
ggggtggggctggagtgcag

SEQ ID NO: 2952 - RNA, 20 nt, synthetic construct
  source 1..20: mol_type = other RNA
ttttgggagtggggtggggc

SEQ ID NO: 2953 - RNA, 20 nt, synthetic construct
  source 1..20: mol_type = other RNA
ttttttttgggagtggggtg

SEQ ID NO: 2954 - RNA, 20 nt, synthetic construct
  source 1..20: mol_type = other RNA
tttttttttgggagtggggt

SEQ ID NO: 2955 - RNA, 20 nt, synthetic construct
  source 1..20: mol_type = other RNA
ttttttttttgggagtgggg

SEQ ID NO: 2956 - RNA, 20 nt, synthetic construct
  source 1..20: mol_type = other RNA
tggttttttttttgggagtg

SEQ ID NO: 2957 - RNA, 20 nt, synthetic construct
  source 1..20: mol_type = other RNA
ttggttttttttttgggagt

SEQ ID NO: 2958 - RNA, 20 nt, synthetic construct
  source 1..20: mol_type = other RNA
tttggttttttttttgggag

SEQ ID NO: 2959 - RNA, 20 nt, synthetic construct
  source 1..20: mol_type = other RNA
tgttttttggtttttttttt

SEQ ID NO: 2960 - RNA, 20 nt, synthetic construct
  source 1..20: mol_type = other RNA
ttgttttttggttttttttt

SEQ ID NO: 2961 - RNA, 20 nt, synthetic construct
  source 1..20: mol_type = other RNA
accaaaaaacaaaaaactaa

SEQ ID NO: 2962 - RNA, 20 nt, synthetic construct
  source 1..20: mol_type = other RNA
acctttagttttttgttttt

SEQ ID NO: 2963 - RNA, 20 nt, synthetic construct
  source 1..20: mol_type = other RNA
cagcatttgtttttctaaag

SEQ ID NO: 2964 - RNA, 20 nt, synthetic construct
  source 1..20: mol_type = other RNA
gaactagctattctactcca

SEQ ID NO: 2965 - RNA, 20 nt, synthetic construct
  source 1..20: mol_type = other RNA
tttctcttgggtatgtgcct

SEQ ID NO: 2966 - RNA, 20 nt, synthetic construct
  source 1..20: mol_type = other RNA
tgtatgtattcgtttctctt

SEQ ID NO: 2967 - RNA, 20 nt, synthetic construct
  source 1..20: mol_type = other RNA
atgtatgtattcgtttctct

SEQ ID NO: 2968 - RNA, 20 nt, synthetic construct
  source 1..20: mol_type = other RNA
catacattcacacaaaaact

SEQ ID NO: 2969 - RNA, 20 nt, synthetic construct
  source 1..20: mol_type = other RNA
aacttggacacatatgttca

SEQ ID NO: 2970 - RNA, 20 nt, synthetic construct
  source 1..20: mol_type = other RNA
acaatcatttgtccatcaac

SEQ ID NO: 2971 - RNA, 20 nt, synthetic construct
  source 1..20: mol_type = other RNA
tttgtccatcaactggtgaa

SEQ ID NO: 2972 - RNA, 20 nt, synthetic construct
  source 1..20: mol_type = other RNA
tttatccattcaccagttga

SEQ ID NO: 2973 - RNA, 20 nt, synthetic construct
  source 1..20: mol_type = other RNA
tggtgaatggataaacaaaa

SEQ ID NO: 2974 - RNA, 20 nt, synthetic construct
  source 1..20: mol_type = other RNA
aatggtatatatctatataa

SEQ ID NO: 2975 - RNA, 20 nt, synthetic construct
  source 1..20: mol_type = other RNA
gctaagttaaagaaaccagc

SEQ ID NO: 2976 - RNA, 20 nt, synthetic construct
  source 1..20: mol_type = other RNA
ctaagttaaagaaaccagcc

SEQ ID NO: 2977 - RNA, 20 nt, synthetic construct
  source 1..20: mol_type = other RNA
ttaaagaaaccagccgggcg

SEQ ID NO: 2978 - RNA, 20 nt, synthetic construct
  source 1..20: mol_type = other RNA
aagaaaccagccgggcgcgg

SEQ ID NO: 2979 - RNA, 20 nt, synthetic construct
  source 1..20: mol_type = other RNA
cgtgagccaccgcgcccggc

SEQ ID NO: 2980 - RNA, 20 nt, synthetic construct
  source 1..20: mol_type = other RNA
caggcgtgagccaccgcgcc

SEQ ID NO: 2981 - RNA, 20 nt, synthetic construct
  source 1..20: mol_type = other RNA
cgcctgtaaccctagcactt

SEQ ID NO: 2982 - RNA, 20 nt, synthetic construct
  source 1..20: mol_type = other RNA
gcctgtaaccctagcacttt

SEQ ID NO: 2983 - RNA, 20 nt, synthetic construct
  source 1..20: mol_type = other RNA
tgtaaccctagcactttggg

SEQ ID NO: 2984 - RNA, 20 nt, synthetic construct
  source 1..20: mol_type = other RNA
tcccaaagtgctagggttac

SEQ ID NO: 2985 - RNA, 20 nt, synthetic construct
  source 1..20: mol_type = other RNA
cctagcactttgggaggccg

SEQ ID NO: 2986 - RNA, 20 nt, synthetic construct
  source 1..20: mol_type = other RNA
gcactttgggaggccgaggc

SEQ ID NO: 2987 - RNA, 20 nt, synthetic construct
  source 1..20: mol_type = other RNA
cctcggcctcccaaagtgct

SEQ ID NO: 2988 - RNA, 20 nt, synthetic construct
  source 1..20: mol_type = other RNA
ctttgggaggccgaggcagg

SEQ ID NO: 2989 - RNA, 20 nt, synthetic construct
  source 1..20: mol_type = other RNA
gccgaggcaggtggatcacg

SEQ ID NO: 2990 - RNA, 20 nt, synthetic construct
  source 1..20: mol_type = other RNA
ggcaggtggatcacgaggtc

SEQ ID NO: 2991 - RNA, 20 nt, synthetic construct
  source 1..20: mol_type = other RNA
acctcgtgatccacctgcct

SEQ ID NO: 2992 - RNA, 20 nt, synthetic construct
  source 1..20: mol_type = other RNA
tcaggagatcgagaccatcc

SEQ ID NO: 2993 - RNA, 20 nt, synthetic construct
  source 1..20: mol_type = other RNA
tttcactgtgttagccagga

SEQ ID NO: 2994 - RNA, 20 nt, synthetic construct
  source 1..20: mol_type = other RNA
ggggtttcactgtgttagcc

SEQ ID NO: 2995 - RNA, 20 nt, synthetic construct
  source 1..20: mol_type = other RNA
ttgtatttttagtagagatg

SEQ ID NO: 2996 - RNA, 20 nt, synthetic construct
  source 1..20: mol_type = other RNA
tttgtatttttagtagagat

SEQ ID NO: 2997 - RNA, 20 nt, synthetic construct
  source 1..20: mol_type = other RNA
ttttgtatttttagtagaga

SEQ ID NO: 2998 - RNA, 20 nt, synthetic construct
  source 1..20: mol_type = other RNA
taaaaatacaaaaaattagc

SEQ ID NO: 2999 - RNA, 20 nt, synthetic construct
  source 1..20: mol_type = other RNA
aaaaatacaaaaaattagcc

SEQ ID NO: 3000 - RNA, 20 nt, synthetic construct
  source 1..20: mol_type = other RNA
tacaaaaaattagccgggtg

SEQ ID NO: 3001 - RNA, 20 nt, synthetic construct
  source 1..20: mol_type = other RNA
aaaaaattagccgggtgtgg

SEQ ID NO: 3002 - RNA, 20 nt, synthetic construct
  source 1..20: mol_type = other RNA
aaattagccgggtgtggtgg

SEQ ID NO: 3003 - RNA, 20 nt, synthetic construct
  source 1..20: mol_type = other RNA
aattagccgggtgtggtggc

SEQ ID NO: 3004 - RNA, 20 nt, synthetic construct
  source 1..20: mol_type = other RNA
caggcgcccgccaccacacc

SEQ ID NO: 3005 - RNA, 20 nt, synthetic construct
  source 1..20: mol_type = other RNA
gcgcctgtagtcccagctac

SEQ ID NO: 3006 - RNA, 20 nt, synthetic construct
  source 1..20: mol_type = other RNA
cgcctgtagtcccagctact

SEQ ID NO: 3007 - RNA, 20 nt, synthetic construct
  source 1..20: mol_type = other RNA
gcctgtagtcccagctactg

SEQ ID NO: 3008 - RNA, 20 nt, synthetic construct
  source 1..20: mol_type = other RNA
tgtagtcccagctactgggg

SEQ ID NO: 3009 - RNA, 20 nt, synthetic construct
  source 1..20: mol_type = other RNA
tccccagtagctgggactac

SEQ ID NO: 3010 - RNA, 20 nt, synthetic construct
  source 1..20: mol_type = other RNA
cccagctactggggaggctg

SEQ ID NO: 3011 - RNA, 20 nt, synthetic construct
  source 1..20: mol_type = other RNA
gctactggggaggctgaggc

SEQ ID NO: 3012 - RNA, 20 nt, synthetic construct
  source 1..20: mol_type = other RNA
cctcagcctccccagtagct

SEQ ID NO: 3013 - RNA, 20 nt, synthetic construct
  source 1..20: mol_type = other RNA
gcctcagcctccccagtagc

SEQ ID NO: 3014 - RNA, 20 nt, synthetic construct
  source 1..20: mol_type = other RNA
gggaggctgaggcaggagaa

SEQ ID NO: 3015 - RNA, 20 nt, synthetic construct
  source 1..20: mol_type = other RNA
caggagaatggcgtgaaccc

SEQ ID NO: 3016 - RNA, 20 nt, synthetic construct
  source 1..20: mol_type = other RNA
gagaatggcgtgaacccagg

SEQ ID NO: 3017 - RNA, 20 nt, synthetic construct
  source 1..20: mol_type = other RNA
aatggcgtgaacccaggagg

SEQ ID NO: 3018 - RNA, 20 nt, synthetic construct
  source 1..20: mol_type = other RNA
atggcgtgaacccaggaggc

SEQ ID NO: 3019 - RNA, 20 nt, synthetic construct
  source 1..20: mol_type = other RNA
tggcgtgaacccaggaggcg

SEQ ID NO: 3020 - RNA, 20 nt, synthetic construct
  source 1..20: mol_type = other RNA
cactgcaagccccgcctcct

SEQ ID NO: 3021 - RNA, 20 nt, synthetic construct
  source 1..20: mol_type = other RNA
tcactgcaagccccgcctcc

SEQ ID NO: 3022 - RNA, 20 nt, synthetic construct
  source 1..20: mol_type = other RNA
ggagtgcagtggtgcaatct

SEQ ID NO: 3023 - RNA, 20 nt, synthetic construct
  source 1..20: mol_type = other RNA
gcaccactgcactccagcct

SEQ ID NO: 3024 - RNA, 20 nt, synthetic construct
  source 1..20: mol_type = other RNA
tcgcctaggctggagtgcag

SEQ ID NO: 3025 - RNA, 20 nt, synthetic construct
  source 1..20: mol_type = other RNA
tctggctctgtcgcctaggc

SEQ ID NO: 3026 - RNA, 20 nt, synthetic construct
  source 1..20: mol_type = other RNA
ggagtctggctctgtcgcct

SEQ ID NO: 3027 - RNA, 20 nt, synthetic construct
  source 1..20: mol_type = other RNA
ttttgtttttgagaggagtc

SEQ ID NO: 3028 - RNA, 20 nt, synthetic construct
  source 1..20: mol_type = other RNA
tgttttgttttgtttttgag

SEQ ID NO: 3029 - RNA, 20 nt, synthetic construct
  source 1..20: mol_type = other RNA
cagatacaaaagactacaca

SEQ ID NO: 3030 - RNA, 20 nt, synthetic construct
  source 1..20: mol_type = other RNA
actacacatggtatgagacc

SEQ ID NO: 3031 - RNA, 20 nt, synthetic construct
  source 1..20: mol_type = other RNA
acatggtatgagaccaggac

SEQ ID NO: 3032 - RNA, 20 nt, synthetic construct
  source 1..20: mol_type = other RNA
catggtatgagaccaggaca

SEQ ID NO: 3033 - RNA, 20 nt, synthetic construct
  source 1..20: mol_type = other RNA
gagaccaggacagggaaatc

SEQ ID NO: 3034 - RNA, 20 nt, synthetic construct
  source 1..20: mol_type = other RNA
gtctccagatttccctgtcc

SEQ ID NO: 3035 - RNA, 20 nt, synthetic construct
  source 1..20: mol_type = other RNA
ggagacagaaagtagattag

SEQ ID NO: 3036 - RNA, 20 nt, synthetic construct
  source 1..20: mol_type = other RNA
aaagtagattagtggttgtc

SEQ ID NO: 3037 - RNA, 20 nt, synthetic construct
  source 1..20: mol_type = other RNA
aagtagattagtggttgtca

SEQ ID NO: 3038 - RNA, 20 nt, synthetic construct
  source 1..20: mol_type = other RNA
agtagattagtggttgtcag

SEQ ID NO: 3039 - RNA, 20 nt, synthetic construct
  source 1..20: mol_type = other RNA
gattagtggttgtcaggggt

SEQ ID NO: 3040 - RNA, 20 nt, synthetic construct
  source 1..20: mol_type = other RNA
attagtggttgtcaggggtt

SEQ ID NO: 3041 - RNA, 20 nt, synthetic construct
  source 1..20: mol_type = other RNA
ggttgtcaggggttgggatg

SEQ ID NO: 3042 - RNA, 20 nt, synthetic construct
  source 1..20: mol_type = other RNA
gttgtcaggggttgggatgt

SEQ ID NO: 3043 - RNA, 20 nt, synthetic construct
  source 1..20: mol_type = other RNA
ggttgggatgtgggtgagaa

SEQ ID NO: 3044 - RNA, 20 nt, synthetic construct
  source 1..20: mol_type = other RNA
gtatgtacccagtctctcct

SEQ ID NO: 3045 - RNA, 20 nt, synthetic construct
  source 1..20: mol_type = other RNA
tatgtacccagtctctcctt

SEQ ID NO: 3046 - RNA, 20 nt, synthetic construct
  source 1..20: mol_type = other RNA
atgtacccagtctctccttg

SEQ ID NO: 3047 - RNA, 20 nt, synthetic construct
  source 1..20: mol_type = other RNA
caacaccccaaggagagact

SEQ ID NO: 3048 - RNA, 20 nt, synthetic construct
  source 1..20: mol_type = other RNA
tcaacaccccaaggagagac

SEQ ID NO: 3049 - RNA, 20 nt, synthetic construct
  source 1..20: mol_type = other RNA
agaatattttcaacacccca

SEQ ID NO: 3050 - RNA, 20 nt, synthetic construct
  source 1..20: mol_type = other RNA
ttttagtatattcacagctg

SEQ ID NO: 3051 - RNA, 20 nt, synthetic construct
  source 1..20: mol_type = other RNA
accactaaactgtacctttt

SEQ ID NO: 3052 - RNA, 20 nt, synthetic construct
  source 1..20: mol_type = other RNA
acctaaaaggtacagtttag

SEQ ID NO: 3053 - RNA, 20 nt, synthetic construct
  source 1..20: mol_type = other RNA
taccttttaggtgaatttta

SEQ ID NO: 3054 - RNA, 20 nt, synthetic construct
  source 1..20: mol_type = other RNA
taccataaaattcacctaaa

SEQ ID NO: 3055 - RNA, 20 nt, synthetic construct
  source 1..20: mol_type = other RNA
atggtatgtgaaatatatct

SEQ ID NO: 3056 - RNA, 20 nt, synthetic construct
  source 1..20: mol_type = other RNA
tatgtgaaatatatctcggc

SEQ ID NO: 3057 - RNA, 20 nt, synthetic construct
  source 1..20: mol_type = other RNA
atgtgaaatatatctcggcc

SEQ ID NO: 3058 - RNA, 20 nt, synthetic construct
  source 1..20: mol_type = other RNA
aaatatatctcggccgggcg

SEQ ID NO: 3059 - RNA, 20 nt, synthetic construct
  source 1..20: mol_type = other RNA
tatatctcggccgggcgtgg

SEQ ID NO: 3060 - RNA, 20 nt, synthetic construct
  source 1..20: mol_type = other RNA
caggcatgagccaccacgcc

SEQ ID NO: 3061 - RNA, 20 nt, synthetic construct
  source 1..20: mol_type = other RNA
tgcctgtaatcccagcactt

SEQ ID NO: 3062 - RNA, 20 nt, synthetic construct
  source 1..20: mol_type = other RNA
gcctgtaatcccagcacttt

SEQ ID NO: 3063 - RNA, 20 nt, synthetic construct
  source 1..20: mol_type = other RNA
tgtaatcccagcactttggg

SEQ ID NO: 3064 - RNA, 20 nt, synthetic construct
  source 1..20: mol_type = other RNA
tcccaaagtgctgggattac

SEQ ID NO: 3065 - RNA, 20 nt, synthetic construct
  source 1..20: mol_type = other RNA
cccagcactttgggaggccg

SEQ ID NO: 3066 - RNA, 20 nt, synthetic construct
  source 1..20: mol_type = other RNA
cctcggcctcccaaagtgct

SEQ ID NO: 3067 - RNA, 20 nt, synthetic construct
  source 1..20: mol_type = other RNA
gcctcggcctcccaaagtgc

SEQ ID NO: 3068 - RNA, 20 nt, synthetic construct
  source 1..20: mol_type = other RNA
ggaggccgaggcaaatcacg

SEQ ID NO: 3069 - RNA, 20 nt, synthetic construct
  source 1..20: mol_type = other RNA
ccgaggcaaatcacgaggtc

SEQ ID NO: 3070 - RNA, 20 nt, synthetic construct
  source 1..20: mol_type = other RNA
cctgacctcgtgatttgcct

SEQ ID NO: 3071 - RNA, 20 nt, synthetic construct
  source 1..20: mol_type = other RNA
tcaggagatcgagaccatcc

SEQ ID NO: 3072 - RNA, 20 nt, synthetic construct
  source 1..20: mol_type = other RNA
cgagaccatcctggctaaca

SEQ ID NO: 3073 - RNA, 20 nt, synthetic construct
  source 1..20: mol_type = other RNA
tttcaccatgttagccagga

SEQ ID NO: 3074 - RNA, 20 nt, synthetic construct
  source 1..20: mol_type = other RNA
ggagtttcaccatgttagcc

SEQ ID NO: 3075 - RNA, 20 nt, synthetic construct
  source 1..20: mol_type = other RNA
tttgtattttttagtagaga

SEQ ID NO: 3076 - RNA, 20 nt, synthetic construct
  source 1..20: mol_type = other RNA
aaaaaatacaaaaaattagc

SEQ ID NO: 3077 - RNA, 20 nt, synthetic construct
  source 1..20: mol_type = other RNA
tacaaaaaattagctggcca

SEQ ID NO: 3078 - RNA, 20 nt, synthetic construct
  source 1..20: mol_type = other RNA
aaaaaattagctggccatgg

SEQ ID NO: 3079 - RNA, 20 nt, synthetic construct
  source 1..20: mol_type = other RNA
aaattagctggccatggtgg

SEQ ID NO: 3080 - RNA, 20 nt, synthetic construct
  source 1..20: mol_type = other RNA
aattagctggccatggtggt

SEQ ID NO: 3081 - RNA, 20 nt, synthetic construct
  source 1..20: mol_type = other RNA
actacaggtgcccaccacca

SEQ ID NO: 3082 - RNA, 20 nt, synthetic construct
  source 1..20: mol_type = other RNA
cacctgtagtcccagctact

SEQ ID NO: 3083 - RNA, 20 nt, synthetic construct
  source 1..20: mol_type = other RNA
acctgtagtcccagctactc

SEQ ID NO: 3084 - RNA, 20 nt, synthetic construct
  source 1..20: mol_type = other RNA
tcccgagtagctgggactac

SEQ ID NO: 3085 - RNA, 20 nt, synthetic construct
  source 1..20: mol_type = other RNA
cccagctactcgggacactg

SEQ ID NO: 3086 - RNA, 20 nt, synthetic construct
  source 1..20: mol_type = other RNA
gctactcgggacactgaggc

SEQ ID NO: 3087 - RNA, 20 nt, synthetic construct
  source 1..20: mol_type = other RNA
cctcagtgtcccgagtagct

SEQ ID NO: 3088 - RNA, 20 nt, synthetic construct
  source 1..20: mol_type = other RNA
gcctcagtgtcccgagtagc

SEQ ID NO: 3089 - RNA, 20 nt, synthetic construct
  source 1..20: mol_type = other RNA
gagaattgcttgaacccaga

SEQ ID NO: 3090 - RNA, 20 nt, synthetic construct
  source 1..20: mol_type = other RNA
aattgcttgaacccagaagg

SEQ ID NO: 3091 - RNA, 20 nt, synthetic construct
  source 1..20: mol_type = other RNA
tgcttgaacccagaaggcgg

SEQ ID NO: 3092 - RNA, 20 nt, synthetic construct
  source 1..20: mol_type = other RNA
cactgcaaccaccgccttct

SEQ ID NO: 3093 - RNA, 20 nt, synthetic construct
  source 1..20: mol_type = other RNA
tcactgcaaccaccgccttc

SEQ ID NO: 3094 - RNA, 20 nt, synthetic construct
  source 1..20: mol_type = other RNA
tgcagtgagtggcgcgatct

SEQ ID NO: 3095 - RNA, 20 nt, synthetic construct
  source 1..20: mol_type = other RNA
ctcgctcggggcggaagtgg

SEQ ID NO: 3096 - RNA, 20 nt, synthetic construct
  source 1..20: mol_type = other RNA
cctctcgctcggggcggaag

SEQ ID NO: 3097 - RNA, 20 nt, synthetic construct
  source 1..20: mol_type = other RNA
cgccccgagcgagaggctag

SEQ ID NO: 3098 - RNA, 20 nt, synthetic construct
  source 1..20: mol_type = other RNA
ctctagcctctcgctcgggg

SEQ ID NO: 3099 - RNA, 20 nt, synthetic construct
  source 1..20: mol_type = other RNA
cgcctctagcctctcgctcg

SEQ ID NO: 3100 - RNA, 20 nt, synthetic construct
  source 1..20: mol_type = other RNA
tcgcctctagcctctcgctc

SEQ ID NO: 3101 - RNA, 20 nt, synthetic construct
  source 1..20: mol_type = other RNA
ctcgcctctagcctctcgct

SEQ ID NO: 3102 - RNA, 20 nt, synthetic construct
  source 1..20: mol_type = other RNA
gagaggctagaggcgagagg

SEQ ID NO: 3103 - RNA, 20 nt, synthetic construct
  source 1..20: mol_type = other RNA
agaggctagaggcgagaggc

SEQ ID NO: 3104 - RNA, 20 nt, synthetic construct
  source 1..20: mol_type = other RNA
gaggctagaggcgagaggcg

SEQ ID NO: 3105 - RNA, 20 nt, synthetic construct
  source 1..20: mol_type = other RNA
aggctagaggcgagaggcgg

SEQ ID NO: 3106 - RNA, 20 nt, synthetic construct
  source 1..20: mol_type = other RNA
ctagaggcgagaggcggggg

SEQ ID NO: 3107 - RNA, 20 nt, synthetic construct
  source 1..20: mol_type = other RNA
gaggcgagaggcgggggagg

SEQ ID NO: 3108 - RNA, 20 nt, synthetic construct
  source 1..20: mol_type = other RNA
aggcgagaggcgggggaggc

SEQ ID NO: 3109 - RNA, 20 nt, synthetic construct
  source 1..20: mol_type = other RNA
cgagaggcgggggaggcggg

SEQ ID NO: 3110 - RNA, 20 nt, synthetic construct
  source 1..20: mol_type = other RNA
gagaggcgggggaggcggga

SEQ ID NO: 3111 - RNA, 20 nt, synthetic construct
  source 1..20: mol_type = other RNA
gggaggcgggagggaccctg

SEQ ID NO: 3112 - RNA, 20 nt, synthetic construct
  source 1..20: mol_type = other RNA
gcgggagggaccctgcggac

SEQ ID NO: 3113 - RNA, 20 nt, synthetic construct
  source 1..20: mol_type = other RNA
cgggagggaccctgcggaca

SEQ ID NO: 3114 - RNA, 20 nt, synthetic construct
  source 1..20: mol_type = other RNA
ctgcggacagggcacgagtc

SEQ ID NO: 3115 - RNA, 20 nt, synthetic construct
  source 1..20: mol_type = other RNA
tgcggacagggcacgagtcc

SEQ ID NO: 3116 - RNA, 20 nt, synthetic construct
  source 1..20: mol_type = other RNA
ggactcgtgccctgtccgca

SEQ ID NO: 3117 - RNA, 20 nt, synthetic construct
  source 1..20: mol_type = other RNA
cggactcgtgccctgtccgc

SEQ ID NO: 3118 - RNA, 20 nt, synthetic construct
  source 1..20: mol_type = other RNA
cagggcacgagtccgggtct

SEQ ID NO: 3119 - RNA, 20 nt, synthetic construct
  source 1..20: mol_type = other RNA
ggcacgagtccgggtctcgg

SEQ ID NO: 3120 - RNA, 20 nt, synthetic construct
  source 1..20: mol_type = other RNA
acgagtccgggtctcggagg

SEQ ID NO: 3121 - RNA, 20 nt, synthetic construct
  source 1..20: mol_type = other RNA
gtccgggtctcggaggaggt

SEQ ID NO: 3122 - RNA, 20 nt, synthetic construct
  source 1..20: mol_type = other RNA
cgccgacctcctccgagacc

SEQ ID NO: 3123 - RNA, 20 nt, synthetic construct
  source 1..20: mol_type = other RNA
ggaggtcggcgactgccgcg

SEQ ID NO: 3124 - RNA, 20 nt, synthetic construct
  source 1..20: mol_type = other RNA
gaggtcggcgactgccgcgt

SEQ ID NO: 3125 - RNA, 20 nt, synthetic construct
  source 1..20: mol_type = other RNA
ggcgcgagcagagcctgcgc

SEQ ID NO: 3126 - RNA, 20 nt, synthetic construct
  source 1..20: mol_type = other RNA
gcgagcagagcctgcgccgg

SEQ ID NO: 3127 - RNA, 20 nt, synthetic construct
  source 1..20: mol_type = other RNA
cagagcctgcgccggcggag

SEQ ID NO: 3128 - RNA, 20 nt, synthetic construct
  source 1..20: mol_type = other RNA
ctgcgccggcggagaggctc

SEQ ID NO: 3129 - RNA, 20 nt, synthetic construct
  source 1..20: mol_type = other RNA
ctgagcctctccgccggcgc

SEQ ID NO: 3130 - RNA, 20 nt, synthetic construct
  source 1..20: mol_type = other RNA
cggggcctgagcctctccgc

SEQ ID NO: 3131 - RNA, 20 nt, synthetic construct
  source 1..20: mol_type = other RNA
ggctcaggccccgcacgatc

SEQ ID NO: 3132 - RNA, 20 nt, synthetic construct
  source 1..20: mol_type = other RNA
gctcaggccccgcacgatcc

SEQ ID NO: 3133 - RNA, 20 nt, synthetic construct
  source 1..20: mol_type = other RNA
ctcaggccccgcacgatccg

SEQ ID NO: 3134 - RNA, 20 nt, synthetic construct
  source 1..20: mol_type = other RNA
gcacgatccggggagagcgc

SEQ ID NO: 3135 - RNA, 20 nt, synthetic construct
  source 1..20: mol_type = other RNA
cgctctccccggatcgtgcg

SEQ ID NO: 3136 - RNA, 20 nt, synthetic construct
  source 1..20: mol_type = other RNA
gcgctctccccggatcgtgc

SEQ ID NO: 3137 - RNA, 20 nt, synthetic construct
  source 1..20: mol_type = other RNA
agcgctctccccggatcgtg

SEQ ID NO: 3138 - RNA, 20 nt, synthetic construct
  source 1..20: mol_type = other RNA
cggggagagcgctggcgctg

SEQ ID NO: 3139 - RNA, 20 nt, synthetic construct
  source 1..20: mol_type = other RNA
cgcagcgccagcgctctccc

SEQ ID NO: 3140 - RNA, 20 nt, synthetic construct
  source 1..20: mol_type = other RNA
cttggcgtgggggcggggcg

SEQ ID NO: 3141 - RNA, 20 nt, synthetic construct
  source 1..20: mol_type = other RNA
gcccccacgccaagccctgt

SEQ ID NO: 3142 - RNA, 20 nt, synthetic construct
  source 1..20: mol_type = other RNA
cagggcttggcgtgggggcg

SEQ ID NO: 3143 - RNA, 20 nt, synthetic construct
  source 1..20: mol_type = other RNA
acagggcttggcgtgggggc

SEQ ID NO: 3144 - RNA, 20 nt, synthetic construct
  source 1..20: mol_type = other RNA
gacagggcttggcgtggggg

SEQ ID NO: 3145 - RNA, 20 nt, synthetic construct
  source 1..20: mol_type = other RNA
acgccaagccctgtcggccg

SEQ ID NO: 3146 - RNA, 20 nt, synthetic construct
  source 1..20: mol_type = other RNA
ggccgacagggcttggcgtg

SEQ ID NO: 3147 - RNA, 20 nt, synthetic construct
  source 1..20: mol_type = other RNA
cggccgacagggcttggcgt

SEQ ID NO: 3148 - RNA, 20 nt, synthetic construct
  source 1..20: mol_type = other RNA
acggccgacagggcttggcg

SEQ ID NO: 3149 - RNA, 20 nt, synthetic construct
  source 1..20: mol_type = other RNA
tccccacggccgacagggct

SEQ ID NO: 3150 - RNA, 20 nt, synthetic construct
  source 1..20: mol_type = other RNA
tactttccccacggccgaca

SEQ ID NO: 3151 - RNA, 20 nt, synthetic construct
  source 1..20: mol_type = other RNA
gtactttccccacggccgac

SEQ ID NO: 3152 - RNA, 20 nt, synthetic construct
  source 1..20: mol_type = other RNA
ggggaaagtacctggagcgt

SEQ ID NO: 3153 - RNA, 20 nt, synthetic construct
  source 1..20: mol_type = other RNA
cgctccaggtactttcccca

SEQ ID NO: 3154 - RNA, 20 nt, synthetic construct
  source 1..20: mol_type = other RNA
gcgctgacgtccgacgctcc

SEQ ID NO: 3155 - RNA, 20 nt, synthetic construct
  source 1..20: mol_type = other RNA
cggacgtcagcgcgcagact

SEQ ID NO: 3156 - RNA, 20 nt, synthetic construct
  source 1..20: mol_type = other RNA
gcagactcggcgcccgagcg

SEQ ID NO: 3157 - RNA, 20 nt, synthetic construct
  source 1..20: mol_type = other RNA
gcccgagcgcggcgcgaagt

SEQ ID NO: 3158 - RNA, 20 nt, synthetic construct
  source 1..20: mol_type = other RNA
cgagcgcggcgcgaagtcgg

SEQ ID NO: 3159 - RNA, 20 nt, synthetic construct
  source 1..20: mol_type = other RNA
gccgacttcgcgccgcgctc

SEQ ID NO: 3160 - RNA, 20 nt, synthetic construct
  source 1..20: mol_type = other RNA
cgccgacttcgcgccgcgct

SEQ ID NO: 3161 - RNA, 20 nt, synthetic construct
  source 1..20: mol_type = other RNA
gcggcgcgaagtcggcggcg

SEQ ID NO: 3162 - RNA, 20 nt, synthetic construct
  source 1..20: mol_type = other RNA
gcgcgaagtcggcggcgggg

SEQ ID NO: 3163 - RNA, 20 nt, synthetic construct
  source 1..20: mol_type = other RNA
cgcgaagtcggcggcggggc

SEQ ID NO: 3164 - RNA, 20 nt, synthetic construct
  source 1..20: mol_type = other RNA
gcgaagtcggcggcggggcg

SEQ ID NO: 3165 - RNA, 20 nt, synthetic construct
  source 1..20: mol_type = other RNA
aagtcggcggcggggcgggg

SEQ ID NO: 3166 - RNA, 20 nt, synthetic construct
  source 1..20: mol_type = other RNA
agtcggcggcggggcggggc

SEQ ID NO: 3167 - RNA, 20 nt, synthetic construct
  source 1..20: mol_type = other RNA
gtcggcggcggggcggggcg

SEQ ID NO: 3168 - RNA, 20 nt, synthetic construct
  source 1..20: mol_type = other RNA
gcggggcggggcggggcgct

SEQ ID NO: 3169 - RNA, 20 nt, synthetic construct
  source 1..20: mol_type = other RNA
cggggcggggcggggcgctc

SEQ ID NO: 3170 - RNA, 20 nt, synthetic construct
  source 1..20: mol_type = other RNA
ggggcggggcggggcgctcg

SEQ ID NO: 3171 - RNA, 20 nt, synthetic construct
  source 1..20: mol_type = other RNA
gggcggggcggggcgctcgg

SEQ ID NO: 3172 - RNA, 20 nt, synthetic construct
  source 1..20: mol_type = other RNA
ggcggggcggggcgctcggg

SEQ ID NO: 3173 - RNA, 20 nt, synthetic construct
  source 1..20: mol_type = other RNA
ggggcggggcgctcgggggg

SEQ ID NO: 3174 - RNA, 20 nt, synthetic construct
  source 1..20: mol_type = other RNA
gggcggggcgctcggggggc

SEQ ID NO: 3175 - RNA, 20 nt, synthetic construct
  source 1..20: mol_type = other RNA
ggcggggcgctcggggggcg

SEQ ID NO: 3176 - RNA, 20 nt, synthetic construct
  source 1..20: mol_type = other RNA
ggcgctcggggggcggggct

SEQ ID NO: 3177 - RNA, 20 nt, synthetic construct
  source 1..20: mol_type = other RNA
gcgctcggggggcggggctc

SEQ ID NO: 3178 - RNA, 20 nt, synthetic construct
  source 1..20: mol_type = other RNA
cgctcggggggcggggctcg

SEQ ID NO: 3179 - RNA, 20 nt, synthetic construct
  source 1..20: mol_type = other RNA
gggcggggctcggggtgccc

SEQ ID NO: 3180 - RNA, 20 nt, synthetic construct
  source 1..20: mol_type = other RNA
cggggctcggggtgcccagg

SEQ ID NO: 3181 - RNA, 20 nt, synthetic construct
  source 1..20: mol_type = other RNA
ggggctcggggtgcccaggt

SEQ ID NO: 3182 - RNA, 20 nt, synthetic construct
  source 1..20: mol_type = other RNA
gctcggggtgcccaggtggg

SEQ ID NO: 3183 - RNA, 20 nt, synthetic construct
  source 1..20: mol_type = other RNA
ctcggggtgcccaggtggga

SEQ ID NO: 3184 - RNA, 20 nt, synthetic construct
  source 1..20: mol_type = other RNA
tcggggtgcccaggtgggag

SEQ ID NO: 3185 - RNA, 20 nt, synthetic construct
  source 1..20: mol_type = other RNA
cggggtgcccaggtgggagg

SEQ ID NO: 3186 - RNA, 20 nt, synthetic construct
  source 1..20: mol_type = other RNA
ggtgcccaggtgggaggggg

SEQ ID NO: 3187 - RNA, 20 nt, synthetic construct
  source 1..20: mol_type = other RNA
gtgcccaggtgggagggggc

SEQ ID NO: 3188 - RNA, 20 nt, synthetic construct
  source 1..20: mol_type = other RNA
tgcccaggtgggagggggcg

SEQ ID NO: 3189 - RNA, 20 nt, synthetic construct
  source 1..20: mol_type = other RNA
aggtgggagggggcggggcc

SEQ ID NO: 3190 - RNA, 20 nt, synthetic construct
  source 1..20: mol_type = other RNA
ggtgggagggggcggggcca

SEQ ID NO: 3191 - RNA, 20 nt, synthetic construct
  source 1..20: mol_type = other RNA
gtgggagggggcggggccag

SEQ ID NO: 3192 - RNA, 20 nt, synthetic construct
  source 1..20: mol_type = other RNA
tggccccgccccctcccacc

SEQ ID NO: 3193 - RNA, 20 nt, synthetic construct
  source 1..20: mol_type = other RNA
ggcggggccaggggaccacc

SEQ ID NO: 3194 - RNA, 20 nt, synthetic construct
  source 1..20: mol_type = other RNA
ggggccaggggaccacccgg

SEQ ID NO: 3195 - RNA, 20 nt, synthetic construct
  source 1..20: mol_type = other RNA
aggggaccacccggcggccg

SEQ ID NO: 3196 - RNA, 20 nt, synthetic construct
  source 1..20: mol_type = other RNA
acggccgccgggtggtcccc

SEQ ID NO: 3197 - RNA, 20 nt, synthetic construct
  source 1..20: mol_type = other RNA
cagggaccacggccgccggg

SEQ ID NO: 3198 - RNA, 20 nt, synthetic construct
  source 1..20: mol_type = other RNA
gcggccgtggtccctgcgcg

SEQ ID NO: 3199 - RNA, 20 nt, synthetic construct
  source 1..20: mol_type = other RNA
gcgcagggaccacggccgcc

SEQ ID NO: 3200 - RNA, 20 nt, synthetic construct
  source 1..20: mol_type = other RNA
cgcgcagggaccacggccgc

SEQ ID NO: 3201 - RNA, 20 nt, synthetic construct
  source 1..20: mol_type = other RNA
tggtccctgcgcgcggcacg

SEQ ID NO: 3202 - RNA, 20 nt, synthetic construct
  source 1..20: mol_type = other RNA
cgtgccgcgcgcagggacca

SEQ ID NO: 3203 - RNA, 20 nt, synthetic construct
  source 1..20: mol_type = other RNA
ctcacctcgtgccgcgcgca

SEQ ID NO: 3204 - RNA, 20 nt, synthetic construct
  source 1..20: mol_type = other RNA
gctcacctcgtgccgcgcgc

SEQ ID NO: 3205 - RNA, 20 nt, synthetic construct
  source 1..20: mol_type = other RNA
gcacgaggtgagccgcccct

SEQ ID NO: 3206 - RNA, 20 nt, synthetic construct
  source 1..20: mol_type = other RNA
cacgaggtgagccgcccctt

SEQ ID NO: 3207 - RNA, 20 nt, synthetic construct
  source 1..20: mol_type = other RNA
gaagacgcaagcccaagggg

SEQ ID NO: 3208 - RNA, 20 nt, synthetic construct
  source 1..20: mol_type = other RNA
tcggaagacgcaagcccaag

SEQ ID NO: 3209 - RNA, 20 nt, synthetic construct
  source 1..20: mol_type = other RNA
gtcggaagacgcaagcccaa

SEQ ID NO: 3210 - RNA, 20 nt, synthetic construct
  source 1..20: mol_type = other RNA
tgtcggaagacgcaagccca

SEQ ID NO: 3211 - RNA, 20 nt, synthetic construct
  source 1..20: mol_type = other RNA
tgcgtcttccgacaagagag

SEQ ID NO: 3212 - RNA, 20 nt, synthetic construct
  source 1..20: mol_type = other RNA
gtcttccgacaagagagagg

SEQ ID NO: 3213 - RNA, 20 nt, synthetic construct
  source 1..20: mol_type = other RNA
ttccgacaagagagaggcgg

SEQ ID NO: 3214 - RNA, 20 nt, synthetic construct
  source 1..20: mol_type = other RNA
aagagagaggcggtggtccg

SEQ ID NO: 3215 - RNA, 20 nt, synthetic construct
  source 1..20: mol_type = other RNA
agagagaggcggtggtccgt

SEQ ID NO: 3216 - RNA, 20 nt, synthetic construct
  source 1..20: mol_type = other RNA
gcggtggtccgtgggtagcg

SEQ ID NO: 3217 - RNA, 20 nt, synthetic construct
  source 1..20: mol_type = other RNA
cggtggtccgtgggtagcgc

SEQ ID NO: 3218 - RNA, 20 nt, synthetic construct
  source 1..20: mol_type = other RNA
ggtggtccgtgggtagcgcg

SEQ ID NO: 3219 - RNA, 20 nt, synthetic construct
  source 1..20: mol_type = other RNA
cgtgggtagcgcggggttac

SEQ ID NO: 3220 - RNA, 20 nt, synthetic construct
  source 1..20: mol_type = other RNA
cagtaaccccgcgctaccca

SEQ ID NO: 3221 - RNA, 20 nt, synthetic construct
  source 1..20: mol_type = other RNA
gtagcgcggggttactggaa

SEQ ID NO: 3222 - RNA, 20 nt, synthetic construct
  source 1..20: mol_type = other RNA
tagcgcggggttactggaat

SEQ ID NO: 3223 - RNA, 20 nt, synthetic construct
  source 1..20: mol_type = other RNA
tactggaatgggactccctg

SEQ ID NO: 3224 - RNA, 20 nt, synthetic construct
  source 1..20: mol_type = other RNA
cttctcaggggacttcctca

SEQ ID NO: 3225 - RNA, 20 nt, synthetic construct
  source 1..20: mol_type = other RNA
acttctcaggggacttcctc

SEQ ID NO: 3226 - RNA, 20 nt, synthetic construct
  source 1..20: mol_type = other RNA
gaagtcccctgagaagtcgc

SEQ ID NO: 3227 - RNA, 20 nt, synthetic construct
  source 1..20: mol_type = other RNA
gcgtgccggcgacttctcag

SEQ ID NO: 3228 - RNA, 20 nt, synthetic construct
  source 1..20: mol_type = other RNA
agcgtgccggcgacttctca

SEQ ID NO: 3229 - RNA, 20 nt, synthetic construct
  source 1..20: mol_type = other RNA
gagcgtgccggcgacttctc

SEQ ID NO: 3230 - RNA, 20 nt, synthetic construct
  source 1..20: mol_type = other RNA
agaaggaaggcggagcgtgc

SEQ ID NO: 3231 - RNA, 20 nt, synthetic construct
  source 1..20: mol_type = other RNA
atgggaagcaagaaggaagg

SEQ ID NO: 3232 - RNA, 20 nt, synthetic construct
  source 1..20: mol_type = other RNA
gaaatgggaagcaagaagga

SEQ ID NO: 3233 - RNA, 20 nt, synthetic construct
  source 1..20: mol_type = other RNA
acgagaaatgggaagcaaga

SEQ ID NO: 3234 - RNA, 20 nt, synthetic construct
  source 1..20: mol_type = other RNA
ctgagaagaaaacgagaaat

SEQ ID NO: 3235 - RNA, 20 nt, synthetic construct
  source 1..20: mol_type = other RNA
gctgagaagaaaacgagaaa

SEQ ID NO: 3236 - RNA, 20 nt, synthetic construct
  source 1..20: mol_type = other RNA
agcactttaaaaaactatga

SEQ ID NO: 3237 - RNA, 20 nt, synthetic construct
  source 1..20: mol_type = other RNA
tattattttaaacatcatct

SEQ ID NO: 3238 - RNA, 20 nt, synthetic construct
  source 1..20: mol_type = other RNA
catcatctaggtcagattag

SEQ ID NO: 3239 - RNA, 20 nt, synthetic construct
  source 1..20: mol_type = other RNA
ttagcggcctgtgaccaact

SEQ ID NO: 3240 - RNA, 20 nt, synthetic construct
  source 1..20: mol_type = other RNA
tttgtttccaagttggtcac

SEQ ID NO: 3241 - RNA, 20 nt, synthetic construct
  source 1..20: mol_type = other RNA
tgaggaatttgtttccaagt

SEQ ID NO: 3242 - RNA, 20 nt, synthetic construct
  source 1..20: mol_type = other RNA
ttcctcattcttttctgccc

SEQ ID NO: 3243 - RNA, 20 nt, synthetic construct
  source 1..20: mol_type = other RNA
caccagggcagaaaagaatg

SEQ ID NO: 3244 - RNA, 20 nt, synthetic construct
  source 1..20: mol_type = other RNA
gcttacaggagctgacacca

SEQ ID NO: 3245 - RNA, 20 nt, synthetic construct
  source 1..20: mol_type = other RNA
ggcttacaggagctgacacc

SEQ ID NO: 3246 - RNA, 20 nt, synthetic construct
  source 1..20: mol_type = other RNA
cataaaatctgcaggcttac

SEQ ID NO: 3247 - RNA, 20 nt, synthetic construct
  source 1..20: mol_type = other RNA
ttatttggcataaaatctgc

SEQ ID NO: 3248 - RNA, 20 nt, synthetic construct
  source 1..20: mol_type = other RNA
ttttatgccaaataaaccgc

SEQ ID NO: 3249 - RNA, 20 nt, synthetic construct
  source 1..20: mol_type = other RNA
aaataaaccgctggagcaaa

SEQ ID NO: 3250 - RNA, 20 nt, synthetic construct
  source 1..20: mol_type = other RNA
ttttgctccagcggtttatt

SEQ ID NO: 3251 - RNA, 20 nt, synthetic construct
  source 1..20: mol_type = other RNA
aaccgctggagcaaaaggaa

SEQ ID NO: 3252 - RNA, 20 nt, synthetic construct
  source 1..20: mol_type = other RNA
tgcctttccttttgctccag

SEQ ID NO: 3253 - RNA, 20 nt, synthetic construct
  source 1..20: mol_type = other RNA
gaaaggcagccagcctctcc

SEQ ID NO: 3254 - RNA, 20 nt, synthetic construct
  source 1..20: mol_type = other RNA
agccagcctctcccggaatt

SEQ ID NO: 3255 - RNA, 20 nt, synthetic construct
  source 1..20: mol_type = other RNA
gccagcctctcccggaattt

SEQ ID NO: 3256 - RNA, 20 nt, synthetic construct
  source 1..20: mol_type = other RNA
cctctcccggaatttgggag

SEQ ID NO: 3257 - RNA, 20 nt, synthetic construct
  source 1..20: mol_type = other RNA
tcccaaattccgggagaggc

SEQ ID NO: 3258 - RNA, 20 nt, synthetic construct
  source 1..20: mol_type = other RNA
cctctcccaaattccgggag

SEQ ID NO: 3259 - RNA, 20 nt, synthetic construct
  source 1..20: mol_type = other RNA
gtatccctctcccaaattcc

SEQ ID NO: 3260 - RNA, 20 nt, synthetic construct
  source 1..20: mol_type = other RNA
ggtatccctctcccaaattc

SEQ ID NO: 3261 - RNA, 20 nt, synthetic construct
  source 1..20: mol_type = other RNA
tgtagaacgttttcttaaca

SEQ ID NO: 3262 - RNA, 20 nt, synthetic construct
  source 1..20: mol_type = other RNA
gtacgtttgtttggtaaaag

SEQ ID NO: 3263 - RNA, 20 nt, synthetic construct
  source 1..20: mol_type = other RNA
accaaacaaacgtactagtt

SEQ ID NO: 3264 - RNA, 20 nt, synthetic construct
  source 1..20: mol_type = other RNA
ccaaacaaacgtactagtta

SEQ ID NO: 3265 - RNA, 20 nt, synthetic construct
  source 1..20: mol_type = other RNA
ccctaactagtacgtttgtt

SEQ ID NO: 3266 - RNA, 20 nt, synthetic construct
  source 1..20: mol_type = other RNA
tcttatgaagattatatagc

SEQ ID NO: 3267 - RNA, 20 nt, synthetic construct
  source 1..20: mol_type = other RNA
aatcttcataagaaacgtga

SEQ ID NO: 3268 - RNA, 20 nt, synthetic construct
  source 1..20: mol_type = other RNA
atcttcataagaaacgtgaa

SEQ ID NO: 3269 - RNA, 20 nt, synthetic construct
  source 1..20: mol_type = other RNA
cataagaaacgtgaagggtt

SEQ ID NO: 3270 - RNA, 20 nt, synthetic construct
  source 1..20: mol_type = other RNA
gaaacgtgaagggttaggaa

SEQ ID NO: 3271 - RNA, 20 nt, synthetic construct
  source 1..20: mol_type = other RNA
ttagccgtgctgtccagtat

SEQ ID NO: 3272 - RNA, 20 nt, synthetic construct
  source 1..20: mol_type = other RNA
tagccgtgctgtccagtatt

SEQ ID NO: 3273 - RNA, 20 nt, synthetic construct
  source 1..20: mol_type = other RNA
aatcccaatactggacagca

SEQ ID NO: 3274 - RNA, 20 nt, synthetic construct
  source 1..20: mol_type = other RNA
taaaatttaaatcccaatac

SEQ ID NO: 3275 - RNA, 20 nt, synthetic construct
  source 1..20: mol_type = other RNA
atattaacttaattcctcag

SEQ ID NO: 3276 - RNA, 20 nt, synthetic construct
  source 1..20: mol_type = other RNA
agtggcaccagccacatttc

SEQ ID NO: 3277 - RNA, 20 nt, synthetic construct
  source 1..20: mol_type = other RNA
aaatgtggctggtgccactg

SEQ ID NO: 3278 - RNA, 20 nt, synthetic construct
  source 1..20: mol_type = other RNA
tggcacacctgaaatgtggc

SEQ ID NO: 3279 - RNA, 20 nt, synthetic construct
  source 1..20: mol_type = other RNA
gttatggcacacctgaaatg

SEQ ID NO: 3280 - RNA, 20 nt, synthetic construct
  source 1..20: mol_type = other RNA
aggtgtgccataaccatgta

SEQ ID NO: 3281 - RNA, 20 nt, synthetic construct
  source 1..20: mol_type = other RNA
ccataaccatgtatggctag

SEQ ID NO: 3282 - RNA, 20 nt, synthetic construct
  source 1..20: mol_type = other RNA
ccactagccatacatggtta

SEQ ID NO: 3283 - RNA, 20 nt, synthetic construct
  source 1..20: mol_type = other RNA
tagcagccactagccataca

SEQ ID NO: 3284 - RNA, 20 nt, synthetic construct
  source 1..20: mol_type = other RNA
atcatcgaagacagttcttt

SEQ ID NO: 3285 - RNA, 20 nt, synthetic construct
  source 1..20: mol_type = other RNA
acagttcttttggacagagc

SEQ ID NO: 3286 - RNA, 20 nt, synthetic construct
  source 1..20: mol_type = other RNA
tttggacagagccggccgag

SEQ ID NO: 3287 - RNA, 20 nt, synthetic construct
  source 1..20: mol_type = other RNA
gccgagaggattacaatact

SEQ ID NO: 3288 - RNA, 20 nt, synthetic construct
  source 1..20: mol_type = other RNA
ccgagaggattacaatactt

SEQ ID NO: 3289 - RNA, 20 nt, synthetic construct
  source 1..20: mol_type = other RNA
agtattgtaatcctctcggc

SEQ ID NO: 3290 - RNA, 20 nt, synthetic construct
  source 1..20: mol_type = other RNA
cccaagtattgtaatcctct

SEQ ID NO: 3291 - RNA, 20 nt, synthetic construct
  source 1..20: mol_type = other RNA
ttcattattttatgtgatta

SEQ ID NO: 3292 - RNA, 20 nt, synthetic construct
  source 1..20: mol_type = other RNA
tttttttttttttctggcta

SEQ ID NO: 3293 - RNA, 20 nt, synthetic construct
  source 1..20: mol_type = other RNA
ttttttttttttttctggct

SEQ ID NO: 3294 - RNA, 20 nt, synthetic construct
  source 1..20: mol_type = other RNA
agaaaaaaaaaaaaaaaagt

SEQ ID NO: 3295 - RNA, 20 nt, synthetic construct
  source 1..20: mol_type = other RNA
aacttttttttttttttttc

SEQ ID NO: 3296 - RNA, 20 nt, synthetic construct
  source 1..20: mol_type = other RNA
aaaaaaaaaaaagttggcta

SEQ ID NO: 3297 - RNA, 20 nt, synthetic construct
  source 1..20: mol_type = other RNA
atagtatgatttagagatac

SEQ ID NO: 3298 - RNA, 20 nt, synthetic construct
  source 1..20: mol_type = other RNA
gacattgtggggtctttcgg

SEQ ID NO: 3299 - RNA, 20 nt, synthetic construct
  source 1..20: mol_type = other RNA
aaagaccccacaatgtctaa

SEQ ID NO: 3300 - RNA, 20 nt, synthetic construct
  source 1..20: mol_type = other RNA
tagacattgtggggtctttc

SEQ ID NO: 3301 - RNA, 20 nt, synthetic construct
  source 1..20: mol_type = other RNA
ttagacattgtggggtcttt

SEQ ID NO: 3302 - RNA, 20 nt, synthetic construct
  source 1..20: mol_type = other RNA
ccacaatgtctaatggtcct

SEQ ID NO: 3303 - RNA, 20 nt, synthetic construct
  source 1..20: mol_type = other RNA
aaggaccattagacattgtg

SEQ ID NO: 3304 - RNA, 20 nt, synthetic construct
  source 1..20: mol_type = other RNA
caaggaccattagacattgt

SEQ ID NO: 3305 - RNA, 20 nt, synthetic construct
  source 1..20: mol_type = other RNA
ccaaggaccattagacattg

SEQ ID NO: 3306 - RNA, 20 nt, synthetic construct
  source 1..20: mol_type = other RNA
atgacagaatttcagaacca

SEQ ID NO: 3307 - RNA, 20 nt, synthetic construct
  source 1..20: mol_type = other RNA
aatctgattattttgattaa

SEQ ID NO: 3308 - RNA, 20 nt, synthetic construct
  source 1..20: mol_type = other RNA
gattattttgattaaaggca

SEQ ID NO: 3309 - RNA, 20 nt, synthetic construct
  source 1..20: mol_type = other RNA
gaacattcacaggatattct

SEQ ID NO: 3310 - RNA, 20 nt, synthetic construct
  source 1..20: mol_type = other RNA
cgaacattcacaggatattc

SEQ ID NO: 3311 - RNA, 20 nt, synthetic construct
  source 1..20: mol_type = other RNA
agactaatgcgaacattcac

SEQ ID NO: 3312 - RNA, 20 nt, synthetic construct
  source 1..20: mol_type = other RNA
agaacacagtattttttggt

SEQ ID NO: 3313 - RNA, 20 nt, synthetic construct
  source 1..20: mol_type = other RNA
aaaaatactgtgttctacaa

SEQ ID NO: 3314 - RNA, 20 nt, synthetic construct
  source 1..20: mol_type = other RNA
ttgtagaacacagtattttt

SEQ ID NO: 3315 - RNA, 20 nt, synthetic construct
  source 1..20: mol_type = other RNA
aatactgtgttctacaaagg

SEQ ID NO: 3316 - RNA, 20 nt, synthetic construct
  source 1..20: mol_type = other RNA
ccaagtattcagcatctctt

SEQ ID NO: 3317 - RNA, 20 nt, synthetic construct
  source 1..20: mol_type = other RNA
ccaaagagatgctgaatact

SEQ ID NO: 3318 - RNA, 20 nt, synthetic construct
  source 1..20: mol_type = other RNA
aattcatttgtcagcctctc

SEQ ID NO: 3319 - RNA, 20 nt, synthetic construct
  source 1..20: mol_type = other RNA
tttgtcagcctctctggttc

SEQ ID NO: 3320 - RNA, 20 nt, synthetic construct
  source 1..20: mol_type = other RNA
ttgtcagcctctctggttcc

SEQ ID NO: 3321 - RNA, 20 nt, synthetic construct
  source 1..20: mol_type = other RNA
tacagctcccggaaccagag

SEQ ID NO: 3322 - RNA, 20 nt, synthetic construct
  source 1..20: mol_type = other RNA
agataggcaaatacagctcc

SEQ ID NO: 3323 - RNA, 20 nt, synthetic construct
  source 1..20: mol_type = other RNA
tgcactcagcaaactaagat

SEQ ID NO: 3324 - RNA, 20 nt, synthetic construct
  source 1..20: mol_type = other RNA
cagcgaagaatctagaacag

SEQ ID NO: 3325 - RNA, 20 nt, synthetic construct
  source 1..20: mol_type = other RNA
acactggatgcaaatgatgc

SEQ ID NO: 3326 - RNA, 20 nt, synthetic construct
  source 1..20: mol_type = other RNA
catttcaaagaagctcacac

SEQ ID NO: 3327 - RNA, 20 nt, synthetic construct
  source 1..20: mol_type = other RNA
tctttgaaatgcaaatttga

SEQ ID NO: 3328 - RNA, 20 nt, synthetic construct
  source 1..20: mol_type = other RNA
tgtggttaacttcatgtggt

SEQ ID NO: 3329 - RNA, 20 nt, synthetic construct
  source 1..20: mol_type = other RNA
gtgatgtggttaacttcatg

SEQ ID NO: 3330 - RNA, 20 nt, synthetic construct
  source 1..20: mol_type = other RNA
tcactgaaaaaaaagaaaca

SEQ ID NO: 3331 - RNA, 20 nt, synthetic construct
  source 1..20: mol_type = other RNA
acatggaaactgaattcacg

SEQ ID NO: 3332 - RNA, 20 nt, synthetic construct
  source 1..20: mol_type = other RNA
catggaaactgaattcacga

SEQ ID NO: 3333 - RNA, 20 nt, synthetic construct
  source 1..20: mol_type = other RNA
actatgcagttgcatgtgaa

SEQ ID NO: 3334 - RNA, 20 nt, synthetic construct
  source 1..20: mol_type = other RNA
aagactcacctccccctgct

SEQ ID NO: 3335 - RNA, 20 nt, synthetic construct
  source 1..20: mol_type = other RNA
agactcacctccccctgctt

SEQ ID NO: 3336 - RNA, 20 nt, synthetic construct
  source 1..20: mol_type = other RNA
gactcacctccccctgcttg

SEQ ID NO: 3337 - RNA, 20 nt, synthetic construct
  source 1..20: mol_type = other RNA
cagcatccccaagcaggggg

SEQ ID NO: 3338 - RNA, 20 nt, synthetic construct
  source 1..20: mol_type = other RNA
ctgcttggggatgctgaact

SEQ ID NO: 3339 - RNA, 20 nt, synthetic construct
  source 1..20: mol_type = other RNA
gttcagcatccccaagcagg

SEQ ID NO: 3340 - RNA, 20 nt, synthetic construct
  source 1..20: mol_type = other RNA
agttcagcatccccaagcag

SEQ ID NO: 3341 - RNA, 20 nt, synthetic construct
  source 1..20: mol_type = other RNA
aagttcagcatccccaagca

SEQ ID NO: 3342 - RNA, 20 nt, synthetic construct
  source 1..20: mol_type = other RNA
caagttcagcatccccaagc

SEQ ID NO: 3343 - RNA, 20 nt, synthetic construct
  source 1..20: mol_type = other RNA
gatgctgaacttggagagct

SEQ ID NO: 3344 - RNA, 20 nt, synthetic construct
  source 1..20: mol_type = other RNA
gaacttggagagcttggcct

SEQ ID NO: 3345 - RNA, 20 nt, synthetic construct
  source 1..20: mol_type = other RNA
ggagagcttggccttggctc

SEQ ID NO: 3346 - RNA, 20 nt, synthetic construct
  source 1..20: mol_type = other RNA
agcttggccttggctctggc

SEQ ID NO: 3347 - RNA, 20 nt, synthetic construct
  source 1..20: mol_type = other RNA
gccttggctctggcaggctc

SEQ ID NO: 3348 - RNA, 20 nt, synthetic construct
  source 1..20: mol_type = other RNA
gccggagcctgccagagcca

SEQ ID NO: 3349 - RNA, 20 nt, synthetic construct
  source 1..20: mol_type = other RNA
tctggcaggctccggcttgc

SEQ ID NO: 3350 - RNA, 20 nt, synthetic construct
  source 1..20: mol_type = other RNA
gcaggctccggcttgctggc

SEQ ID NO: 3351 - RNA, 20 nt, synthetic construct
  source 1..20: mol_type = other RNA
caggctccggcttgctggca

SEQ ID NO: 3352 - RNA, 20 nt, synthetic construct
  source 1..20: mol_type = other RNA
gggagtccctgccagcaagc

SEQ ID NO: 3353 - RNA, 20 nt, synthetic construct
  source 1..20: mol_type = other RNA
gtgcactgcacatcatacag

SEQ ID NO: 3354 - RNA, 20 nt, synthetic construct
  source 1..20: mol_type = other RNA
cgtgcactgcacatcataca

SEQ ID NO: 3355 - RNA, 20 nt, synthetic construct
  source 1..20: mol_type = other RNA
gcgtgcactgcacatcatac

SEQ ID NO: 3356 - RNA, 20 nt, synthetic construct
  source 1..20: mol_type = other RNA
tccgaagacgacttcagctt

SEQ ID NO: 3357 - RNA, 20 nt, synthetic construct
  source 1..20: mol_type = other RNA
tcctaagctgaagtcgtctt

SEQ ID NO: 3358 - RNA, 20 nt, synthetic construct
  source 1..20: mol_type = other RNA
ttcagcttaggagactcatc

SEQ ID NO: 3359 - RNA, 20 nt, synthetic construct
  source 1..20: mol_type = other RNA
tcagcttaggagactcatca

SEQ ID NO: 3360 - RNA, 20 nt, synthetic construct
  source 1..20: mol_type = other RNA
cagcttaggagactcatcag

SEQ ID NO: 3361 - RNA, 20 nt, synthetic construct
  source 1..20: mol_type = other RNA
actcatcaggggcctgatct

SEQ ID NO: 3362 - RNA, 20 nt, synthetic construct
  source 1..20: mol_type = other RNA
gcctgatcttggccgtccat

SEQ ID NO: 3363 - RNA, 20 nt, synthetic construct
  source 1..20: mol_type = other RNA
gccaatggacggccaagatc

SEQ ID NO: 3364 - RNA, 20 nt, synthetic construct
  source 1..20: mol_type = other RNA
gtccattggcctcacatacg

SEQ ID NO: 3365 - RNA, 20 nt, synthetic construct
  source 1..20: mol_type = other RNA
gcgtatgtgaggccaatgga

SEQ ID NO: 3366 - RNA, 20 nt, synthetic construct
  source 1..20: mol_type = other RNA
attggcctcacatacgcggt

SEQ ID NO: 3367 - RNA, 20 nt, synthetic construct
  source 1..20: mol_type = other RNA
gaccgcgtatgtgaggccaa

SEQ ID NO: 3368 - RNA, 20 nt, synthetic construct
  source 1..20: mol_type = other RNA
agaaaccgaccgcgtatgtg

SEQ ID NO: 3369 - RNA, 20 nt, synthetic construct
  source 1..20: mol_type = other RNA
cggtcggtttctgctggacc

SEQ ID NO: 3370 - RNA, 20 nt, synthetic construct
  source 1..20: mol_type = other RNA
cggtttctgctggaccaggc

SEQ ID NO: 3371 - RNA, 20 nt, synthetic construct
  source 1..20: mol_type = other RNA
ggtttctgctggaccaggct

SEQ ID NO: 3372 - RNA, 20 nt, synthetic construct
  source 1..20: mol_type = other RNA
ccaggctgggttttgaagct

SEQ ID NO: 3373 - RNA, 20 nt, synthetic construct
  source 1..20: mol_type = other RNA
caggctgggttttgaagcta

SEQ ID NO: 3374 - RNA, 20 nt, synthetic construct
  source 1..20: mol_type = other RNA
ctgggttttgaagctaggga

SEQ ID NO: 3375 - RNA, 20 nt, synthetic construct
  source 1..20: mol_type = other RNA
ggttttgaagctagggatgg

SEQ ID NO: 3376 - RNA, 20 nt, synthetic construct
  source 1..20: mol_type = other RNA
gtgtccgctgctgctgtgct

SEQ ID NO: 3377 - RNA, 20 nt, synthetic construct
  source 1..20: mol_type = other RNA
gcggccaagcacagcagcag

SEQ ID NO: 3378 - RNA, 20 nt, synthetic construct
  source 1..20: mol_type = other RNA
ctgtgcttggccgccatggc

SEQ ID NO: 3379 - RNA, 20 nt, synthetic construct
  source 1..20: mol_type = other RNA
tgcttggccgccatggcagg

SEQ ID NO: 3380 - RNA, 20 nt, synthetic construct
  source 1..20: mol_type = other RNA
ccatggcaggtggcctctcc

SEQ ID NO: 3381 - RNA, 20 nt, synthetic construct
  source 1..20: mol_type = other RNA
catggcaggtggcctctcct

SEQ ID NO: 3382 - RNA, 20 nt, synthetic construct
  source 1..20: mol_type = other RNA
ggagaggccacctgccatgg

SEQ ID NO: 3383 - RNA, 20 nt, synthetic construct
  source 1..20: mol_type = other RNA
ccaggagaggccacctgcca

SEQ ID NO: 3384 - RNA, 20 nt, synthetic construct
  source 1..20: mol_type = other RNA
gtggcctctcctgggtctga

SEQ ID NO: 3385 - RNA, 20 nt, synthetic construct
  source 1..20: mol_type = other RNA
tgggccttcagacccaggag

SEQ ID NO: 3386 - RNA, 20 nt, synthetic construct
  source 1..20: mol_type = other RNA
ggaggtgggccttcagaccc

SEQ ID NO: 3387 - RNA, 20 nt, synthetic construct
  source 1..20: mol_type = other RNA
caagtgtgcaatgtggaggt

SEQ ID NO: 3388 - RNA, 20 nt, synthetic construct
  source 1..20: mol_type = other RNA
acaagtgtgcaatgtggagg

SEQ ID NO: 3389 - RNA, 20 nt, synthetic construct
  source 1..20: mol_type = other RNA
caaacaagtgtgcaatgtgg

SEQ ID NO: 3390 - RNA, 20 nt, synthetic construct
  source 1..20: mol_type = other RNA
ggccaaacaagtgtgcaatg

SEQ ID NO: 3391 - RNA, 20 nt, synthetic construct
  source 1..20: mol_type = other RNA
tgttggcagacagcagcctc

SEQ ID NO: 3392 - RNA, 20 nt, synthetic construct
  source 1..20: mol_type = other RNA
gtgttggcagacagcagcct

SEQ ID NO: 3393 - RNA, 20 nt, synthetic construct
  source 1..20: mol_type = other RNA
gccaacaccatctccaagca

SEQ ID NO: 3394 - RNA, 20 nt, synthetic construct
  source 1..20: mol_type = other RNA
accttgcttggagatggtgt

SEQ ID NO: 3395 - RNA, 20 nt, synthetic construct
  source 1..20: mol_type = other RNA
ctcaggaccttgcttggaga

SEQ ID NO: 3396 - RNA, 20 nt, synthetic construct
  source 1..20: mol_type = other RNA
ggctctctcaggaccttgct

SEQ ID NO: 3397 - RNA, 20 nt, synthetic construct
  source 1..20: mol_type = other RNA
cagcacaacagggctctctc

SEQ ID NO: 3398 - RNA, 20 nt, synthetic construct
  source 1..20: mol_type = other RNA
agagccctgttgtgctgagt

SEQ ID NO: 3399 - RNA, 20 nt, synthetic construct
  source 1..20: mol_type = other RNA
tcttccaactcagcacaaca

SEQ ID NO: 3400 - RNA, 20 nt, synthetic construct
  source 1..20: mol_type = other RNA
ttcttccaactcagcacaac

SEQ ID NO: 3401 - RNA, 20 nt, synthetic construct
  source 1..20: mol_type = other RNA
tgagttggaagaagaagaag

SEQ ID NO: 3402 - RNA, 20 nt, synthetic construct
  source 1..20: mol_type = other RNA
agaagaagaagaggaagata

SEQ ID NO: 3403 - RNA, 20 nt, synthetic construct
  source 1..20: mol_type = other RNA
agaagaggaagataaggatg

SEQ ID NO: 3404 - RNA, 20 nt, synthetic construct
  source 1..20: mol_type = other RNA
gaagaggaagataaggatga

SEQ ID NO: 3405 - RNA, 20 nt, synthetic construct
  source 1..20: mol_type = other RNA
aagaggaagataaggatgag

SEQ ID NO: 3406 - RNA, 20 nt, synthetic construct
  source 1..20: mol_type = other RNA
agaggaagataaggatgagg

SEQ ID NO: 3407 - RNA, 20 nt, synthetic construct
  source 1..20: mol_type = other RNA
gaggaagataaggatgaggg

SEQ ID NO: 3408 - RNA, 20 nt, synthetic construct
  source 1..20: mol_type = other RNA
gatgaggggggtcgacacat

SEQ ID NO: 3409 - RNA, 20 nt, synthetic construct
  source 1..20: mol_type = other RNA
atgaggggggtcgacacata

SEQ ID NO: 3410 - RNA, 20 nt, synthetic construct
  source 1..20: mol_type = other RNA
cttttttcattatagttctc

SEQ ID NO: 3411 - RNA, 20 nt, synthetic construct
  source 1..20: mol_type = other RNA
ttttttcattatagttctct

SEQ ID NO: 3412 - RNA, 20 nt, synthetic construct
  source 1..20: mol_type = other RNA
gagcaagtaagcacaggcac

SEQ ID NO: 3413 - RNA, 20 nt, synthetic construct
  source 1..20: mol_type = other RNA
tgtgcttacttgctctctgt

SEQ ID NO: 3414 - RNA, 20 nt, synthetic construct
  source 1..20: mol_type = other RNA
aacagagagcaagtaagcac

SEQ ID NO: 3415 - RNA, 20 nt, synthetic construct
  source 1..20: mol_type = other RNA
tgctctctgttggccgtcag

SEQ ID NO: 3416 - RNA, 20 nt, synthetic construct
  source 1..20: mol_type = other RNA
gctctctgttggccgtcaga

SEQ ID NO: 3417 - RNA, 20 nt, synthetic construct
  source 1..20: mol_type = other RNA
ctctgttggccgtcagaggg

SEQ ID NO: 3418 - RNA, 20 nt, synthetic construct
  source 1..20: mol_type = other RNA
tctgttggccgtcagagggt

SEQ ID NO: 3419 - RNA, 20 nt, synthetic construct
  source 1..20: mol_type = other RNA
gctgggcacccaccctctga

SEQ ID NO: 3420 - RNA, 20 nt, synthetic construct
  source 1..20: mol_type = other RNA
ctatgggctggcagaaggct

SEQ ID NO: 3421 - RNA, 20 nt, synthetic construct
  source 1..20: mol_type = other RNA
actatgggctggcagaaggc

SEQ ID NO: 3422 - RNA, 20 nt, synthetic construct
  source 1..20: mol_type = other RNA
aggcactatgggctggcaga

SEQ ID NO: 3423 - RNA, 20 nt, synthetic construct
  source 1..20: mol_type = other RNA
gtaagagaggcactatgggc

SEQ ID NO: 3424 - RNA, 20 nt, synthetic construct
  source 1..20: mol_type = other RNA
cagagtaagagaggcactat

SEQ ID NO: 3425 - RNA, 20 nt, synthetic construct
  source 1..20: mol_type = other RNA
gcagagtaagagaggcacta

SEQ ID NO: 3426 - RNA, 20 nt, synthetic construct
  source 1..20: mol_type = other RNA
gcctctcttactctgctgca

SEQ ID NO: 3427 - RNA, 20 nt, synthetic construct
  source 1..20: mol_type = other RNA
cctctcttactctgctgcac

SEQ ID NO: 3428 - RNA, 20 nt, synthetic construct
  source 1..20: mol_type = other RNA
ctctcttactctgctgcacg

SEQ ID NO: 3429 - RNA, 20 nt, synthetic construct
  source 1..20: mol_type = other RNA
cccgtgcagcagagtaagag

SEQ ID NO: 3430 - RNA, 20 nt, synthetic construct
  source 1..20: mol_type = other RNA
tgctgcacggggacagctgc

SEQ ID NO: 3431 - RNA, 20 nt, synthetic construct
  source 1..20: mol_type = other RNA
cacggggacagctgctggtg

SEQ ID NO: 3432 - RNA, 20 nt, synthetic construct
  source 1..20: mol_type = other RNA
tgtagtgctacagatagacg

SEQ ID NO: 3433 - RNA, 20 nt, synthetic construct
  source 1..20: mol_type = other RNA
gtagtgctacagatagacga

SEQ ID NO: 3434 - RNA, 20 nt, synthetic construct
  source 1..20: mol_type = other RNA
tgctacagatagacgagggc

SEQ ID NO: 3435 - RNA, 20 nt, synthetic construct
  source 1..20: mol_type = other RNA
agatagacgagggctggttc

SEQ ID NO: 3436 - RNA, 20 nt, synthetic construct
  source 1..20: mol_type = other RNA
gatagacgagggctggttct

SEQ ID NO: 3437 - RNA, 20 nt, synthetic construct
  source 1..20: mol_type = other RNA
tgttcatcgatcttgttcac

SEQ ID NO: 3438 - RNA, 20 nt, synthetic construct
  source 1..20: mol_type = other RNA
atcttgttcacaggagtctg

SEQ ID NO: 3439 - RNA, 20 nt, synthetic construct
  source 1..20: mol_type = other RNA
acaggagtctgaggaacccc

SEQ ID NO: 3440 - RNA, 20 nt, synthetic construct
  source 1..20: mol_type = other RNA
agtctgaggaaccccaggtt

SEQ ID NO: 3441 - RNA, 20 nt, synthetic construct
  source 1..20: mol_type = other RNA
gtctgaggaaccccaggttt

SEQ ID NO: 3442 - RNA, 20 nt, synthetic construct
  source 1..20: mol_type = other RNA
cgttggagttcccaaacctg

SEQ ID NO: 3443 - RNA, 20 nt, synthetic construct
  source 1..20: mol_type = other RNA
tcgttggagttcccaaacct

SEQ ID NO: 3444 - RNA, 20 nt, synthetic construct
  source 1..20: mol_type = other RNA
ctcgttggagttcccaaacc

SEQ ID NO: 3445 - RNA, 20 nt, synthetic construct
  source 1..20: mol_type = other RNA
tccaacgagatgactctgat

SEQ ID NO: 3446 - RNA, 20 nt, synthetic construct
  source 1..20: mol_type = other RNA
tccaatcagagtcatctcgt

SEQ ID NO: 3447 - RNA, 20 nt, synthetic construct
  source 1..20: mol_type = other RNA
cataattgcctaaagtgttc

SEQ ID NO: 3448 - RNA, 20 nt, synthetic construct
  source 1..20: mol_type = other RNA
tgcctaaagtgttctggatc

SEQ ID NO: 3449 - RNA, 20 nt, synthetic construct
  source 1..20: mol_type = other RNA
taaagtgttctggatccggt

SEQ ID NO: 3450 - RNA, 20 nt, synthetic construct
  source 1..20: mol_type = other RNA
aaccggatccagaacacttt

SEQ ID NO: 3451 - RNA, 20 nt, synthetic construct
  source 1..20: mol_type = other RNA
agggggatgaactctccaac

SEQ ID NO: 3452 - RNA, 20 nt, synthetic construct
  source 1..20: mol_type = other RNA
gttcatcccccttgttagtc

SEQ ID NO: 3453 - RNA, 20 nt, synthetic construct
  source 1..20: mol_type = other RNA
ctttctccagactaacaagg

SEQ ID NO: 3454 - RNA, 20 nt, synthetic construct
  source 1..20: mol_type = other RNA
tctttctccagactaacaag

SEQ ID NO: 3455 - RNA, 20 nt, synthetic construct
  source 1..20: mol_type = other RNA
ttctttctccagactaacaa

SEQ ID NO: 3456 - RNA, 20 nt, synthetic construct
  source 1..20: mol_type = other RNA
tttctttctccagactaaca

SEQ ID NO: 3457 - RNA, 20 nt, synthetic construct
  source 1..20: mol_type = other RNA
tgttgtctctaacaatagcg

SEQ ID NO: 3458 - RNA, 20 nt, synthetic construct
  source 1..20: mol_type = other RNA
gttagagacaacagaaacac

SEQ ID NO: 3459 - RNA, 20 nt, synthetic construct
  source 1..20: mol_type = other RNA
aaacaccggagataatcaac

SEQ ID NO: 3460 - RNA, 20 nt, synthetic construct
  source 1..20: mol_type = other RNA
gggcacctgttgattatctc

SEQ ID NO: 3461 - RNA, 20 nt, synthetic construct
  source 1..20: mol_type = other RNA
cccttatcaatcacagagcc

SEQ ID NO: 3462 - RNA, 20 nt, synthetic construct
  source 1..20: mol_type = other RNA
ccttatcaatcacagagcca

SEQ ID NO: 3463 - RNA, 20 nt, synthetic construct
  source 1..20: mol_type = other RNA
cctggctctgtgattgataa

SEQ ID NO: 3464 - RNA, 20 nt, synthetic construct
  source 1..20: mol_type = other RNA
ccctggctctgtgattgata

SEQ ID NO: 3465 - RNA, 20 nt, synthetic construct
  source 1..20: mol_type = other RNA
cattctgcatgtgacaaccc

SEQ ID NO: 3466 - RNA, 20 nt, synthetic construct
  source 1..20: mol_type = other RNA
tcttctgtctgttcagccca

SEQ ID NO: 3467 - RNA, 20 nt, synthetic construct
  source 1..20: mol_type = other RNA
atcttctgtctgttcagccc

SEQ ID NO: 3468 - RNA, 20 nt, synthetic construct
  source 1..20: mol_type = other RNA
acagaagatgcagtcaagtt

SEQ ID NO: 3469 - RNA, 20 nt, synthetic construct
  source 1..20: mol_type = other RNA
aagatgcagtcaagtttggt

SEQ ID NO: 3470 - RNA, 20 nt, synthetic construct
  source 1..20: mol_type = other RNA
tcggccaattcttttagtca

SEQ ID NO: 3471 - RNA, 20 nt, synthetic construct
  source 1..20: mol_type = other RNA
gtggccttgactaaaagaat

SEQ ID NO: 3472 - RNA, 20 nt, synthetic construct
  source 1..20: mol_type = other RNA
ttagtcaaggccaccgtcac

SEQ ID NO: 3473 - RNA, 20 nt, synthetic construct
  source 1..20: mol_type = other RNA
tagtcaaggccaccgtcaca

SEQ ID NO: 3474 - RNA, 20 nt, synthetic construct
  source 1..20: mol_type = other RNA
tctctcactccctgtgacgg

SEQ ID NO: 3475 - RNA, 20 nt, synthetic construct
  source 1..20: mol_type = other RNA
gtttctctcactccctgtga

SEQ ID NO: 3476 - RNA, 20 nt, synthetic construct
  source 1..20: mol_type = other RNA
gagtgagagaaacaagtgag

SEQ ID NO: 3477 - RNA, 20 nt, synthetic construct
  source 1..20: mol_type = other RNA
ctgaaaaccatctaccttgt

SEQ ID NO: 3478 - RNA, 20 nt, synthetic construct
  source 1..20: mol_type = other RNA
tgaaaaccatctaccttgta

SEQ ID NO: 3479 - RNA, 20 nt, synthetic construct
  source 1..20: mol_type = other RNA
agtgagccctacaaggtaga

SEQ ID NO: 3480 - RNA, 20 nt, synthetic construct
  source 1..20: mol_type = other RNA
tctcttcagtgagccctaca

SEQ ID NO: 3481 - RNA, 20 nt, synthetic construct
  source 1..20: mol_type = other RNA
caagaaactcaacaggatga

SEQ ID NO: 3482 - RNA, 20 nt, synthetic construct
  source 1..20: mol_type = other RNA
aagaaatcaagaaactcaac

SEQ ID NO: 3483 - RNA, 20 nt, synthetic construct
  source 1..20: mol_type = other RNA
ctccgtaatgcatttctatc

SEQ ID NO: 3484 - RNA, 20 nt, synthetic construct
  source 1..20: mol_type = other RNA
cagatagaaatgcattacgg

SEQ ID NO: 3485 - RNA, 20 nt, synthetic construct
  source 1..20: mol_type = other RNA
aaccagatagaaatgcatta

SEQ ID NO: 3486 - RNA, 20 nt, synthetic construct
  source 1..20: mol_type = other RNA
tggttcatagacactgcatc

SEQ ID NO: 3487 - RNA, 20 nt, synthetic construct
  source 1..20: mol_type = other RNA
tacagtttaatttgtgtgtg

SEQ ID NO: 3488 - RNA, 20 nt, synthetic construct
  source 1..20: mol_type = other RNA
actcacacaagtgttacatt

SEQ ID NO: 3489 - RNA, 20 nt, synthetic construct
  source 1..20: mol_type = other RNA
cactcacacaagtgttacat

SEQ ID NO: 3490 - RNA, 20 nt, synthetic construct
  source 1..20: mol_type = other RNA
cttgtgtgagtgcagaagtc

SEQ ID NO: 3491 - RNA, 20 nt, synthetic construct
  source 1..20: mol_type = other RNA
gagtgcagaagtctggttcg

SEQ ID NO: 3492 - RNA, 20 nt, synthetic construct
  source 1..20: mol_type = other RNA
aagtctggttcgtggacaaa

SEQ ID NO: 3493 - RNA, 20 nt, synthetic construct
  source 1..20: mol_type = other RNA
tggtgatgacaacaagaaca

SEQ ID NO: 3494 - RNA, 20 nt, synthetic construct
  source 1..20: mol_type = other RNA
cccaaccagacacacaagac

SEQ ID NO: 3495 - RNA, 20 nt, synthetic construct
  source 1..20: mol_type = other RNA
ccagtcttgtgtgtctggtt

SEQ ID NO: 3496 - RNA, 20 nt, synthetic construct
  source 1..20: mol_type = other RNA
accagtcttgtgtgtctggt

SEQ ID NO: 3497 - RNA, 20 nt, synthetic construct
  source 1..20: mol_type = other RNA
tcacaccagtcttgtgtgtc

SEQ ID NO: 3498 - RNA, 20 nt, synthetic construct
  source 1..20: mol_type = other RNA
gactggtgtgatgcacgaag

SEQ ID NO: 3499 - RNA, 20 nt, synthetic construct
  source 1..20: mol_type = other RNA
cgaagtggcctcatgtaaga

SEQ ID NO: 3500 - RNA, 20 nt, synthetic construct
  source 1..20: mol_type = other RNA
ggcctcatgtaagatggagc

SEQ ID NO: 3501 - RNA, 20 nt, synthetic construct
  source 1..20: mol_type = other RNA
tcatgtaagatggagcaggc

SEQ ID NO: 3502 - RNA, 20 nt, synthetic construct
  source 1..20: mol_type = other RNA
tgtaagatggagcaggcagg

SEQ ID NO: 3503 - RNA, 20 nt, synthetic construct
  source 1..20: mol_type = other RNA
tggtcattgagaatgatttc

SEQ ID NO: 3504 - RNA, 20 nt, synthetic construct
  source 1..20: mol_type = other RNA
ggtcattgagaatgatttct

SEQ ID NO: 3505 - RNA, 20 nt, synthetic construct
  source 1..20: mol_type = other RNA
tgatttctgggcttctcaga

SEQ ID NO: 3506 - RNA, 20 nt, synthetic construct
  source 1..20: mol_type = other RNA
aggtattattttgggcatgg

SEQ ID NO: 3507 - RNA, 20 nt, synthetic construct
  source 1..20: mol_type = other RNA
gaggtattattttgggcatg

SEQ ID NO: 3508 - RNA, 20 nt, synthetic construct
  source 1..20: mol_type = other RNA
ggaggtattattttgggcat

SEQ ID NO: 3509 - RNA, 20 nt, synthetic construct
  source 1..20: mol_type = other RNA
aggaggtattattttgggca

SEQ ID NO: 3510 - RNA, 20 nt, synthetic construct
  source 1..20: mol_type = other RNA
gatgcaggaggtattatttt

SEQ ID NO: 3511 - RNA, 20 nt, synthetic construct
  source 1..20: mol_type = other RNA
agatgcaggaggtattattt

SEQ ID NO: 3512 - RNA, 20 nt, synthetic construct
  source 1..20: mol_type = other RNA
catcagccagcagatgcagg

SEQ ID NO: 3513 - RNA, 20 nt, synthetic construct
  source 1..20: mol_type = other RNA
agtcatcagccagcagatgc

SEQ ID NO: 3514 - RNA, 20 nt, synthetic construct
  source 1..20: mol_type = other RNA
caactagagagtcattcctc

SEQ ID NO: 3515 - RNA, 20 nt, synthetic construct
  source 1..20: mol_type = other RNA
gaggaatgactctctagttg

SEQ ID NO: 3516 - RNA, 20 nt, synthetic construct
  source 1..20: mol_type = other RNA
gtgaagacatcttaaaccag

SEQ ID NO: 3517 - RNA, 20 nt, synthetic construct
  source 1..20: mol_type = other RNA
ggtgtttatatttcttgcag

SEQ ID NO: 3518 - RNA, 20 nt, synthetic construct
  source 1..20: mol_type = other RNA
tggtgtttatatttcttgca

SEQ ID NO: 3519 - RNA, 20 nt, synthetic construct
  source 1..20: mol_type = other RNA
gtggtgtttatatttcttgc

SEQ ID NO: 3520 - RNA, 20 nt, synthetic construct
  source 1..20: mol_type = other RNA
taaagtgtttcagcttcttg

SEQ ID NO: 3521 - RNA, 20 nt, synthetic construct
  source 1..20: mol_type = other RNA
taagatactcaaggctaatc

SEQ ID NO: 3522 - RNA, 20 nt, synthetic construct
  source 1..20: mol_type = other RNA
catgcacgctaagatactca

SEQ ID NO: 3523 - RNA, 20 nt, synthetic construct
  source 1..20: mol_type = other RNA
agcatattttccagaagccg

SEQ ID NO: 3524 - RNA, 20 nt, synthetic construct
  source 1..20: mol_type = other RNA
gcatattttccagaagccga

SEQ ID NO: 3525 - RNA, 20 nt, synthetic construct
  source 1..20: mol_type = other RNA
catattttccagaagccgag

SEQ ID NO: 3526 - RNA, 20 nt, synthetic construct
  source 1..20: mol_type = other RNA
gattctttcccctcggcttc

SEQ ID NO: 3527 - RNA, 20 nt, synthetic construct
  source 1..20: mol_type = other RNA
ggggaaagaatccaagatcc

SEQ ID NO: 3528 - RNA, 20 nt, synthetic construct
  source 1..20: mol_type = other RNA
gctatgcagagtaaactctc

SEQ ID NO: 3529 - RNA, 20 nt, synthetic construct
  source 1..20: mol_type = other RNA
gtaatgatgaagacaagcta

SEQ ID NO: 3530 - RNA, 20 nt, synthetic construct
  source 1..20: mol_type = other RNA
ctaaggtaatctaaaacaac

SEQ ID NO: 3531 - RNA, 20 nt, synthetic construct
  source 1..20: mol_type = other RNA
ggaagataattgatgataaa

SEQ ID NO: 3532 - RNA, 20 nt, synthetic construct
  source 1..20: mol_type = other RNA
atcatcaattatcttcctct

SEQ ID NO: 3533 - RNA, 20 nt, synthetic construct
  source 1..20: mol_type = other RNA
atttttcaactgctgccaag

SEQ ID NO: 3534 - RNA, 20 nt, synthetic construct
  source 1..20: mol_type = other RNA
ttatgttttactcaaaagtc

SEQ ID NO: 3535 - RNA, 20 nt, synthetic construct
  source 1..20: mol_type = other RNA
atacaacacttgaactgtgt

SEQ ID NO: 3536 - RNA, 20 nt, synthetic construct
  source 1..20: mol_type = other RNA
tacaacacttgaactgtgtt

SEQ ID NO: 3537 - RNA, 20 nt, synthetic construct
  source 1..20: mol_type = other RNA
tgtcagcgtgttagccactg

SEQ ID NO: 3538 - RNA, 20 nt, synthetic construct
  source 1..20: mol_type = other RNA
cagaatttgaaattccacag

SEQ ID NO: 3539 - RNA, 20 nt, synthetic construct
  source 1..20: mol_type = other RNA
ccgagagttgactctgagag

SEQ ID NO: 3540 - RNA, 20 nt, synthetic construct
  source 1..20: mol_type = other RNA
cactctcagagtcaactctc

SEQ ID NO: 3541 - RNA, 20 nt, synthetic construct
  source 1..20: mol_type = other RNA
ccactctcagagtcaactct

SEQ ID NO: 3542 - RNA, 20 nt, synthetic construct
  source 1..20: mol_type = other RNA
tcttctaataactgtattct

SEQ ID NO: 3543 - RNA, 20 nt, synthetic construct
  source 1..20: mol_type = other RNA
gagctaaaacatctcatttt

SEQ ID NO: 3544 - RNA, 20 nt, synthetic construct
  source 1..20: mol_type = other RNA
gccaagagtgtgaaaacaca

SEQ ID NO: 3545 - RNA, 20 nt, synthetic construct
  source 1..20: mol_type = other RNA
ccaagagtgtgaaaacacat

SEQ ID NO: 3546 - RNA, 20 nt, synthetic construct
  source 1..20: mol_type = other RNA
caagagtgtgaaaacacatg

SEQ ID NO: 3547 - RNA, 20 nt, synthetic construct
  source 1..20: mol_type = other RNA
aagagtgtgaaaacacatgg

SEQ ID NO: 3548 - RNA, 20 nt, synthetic construct
  source 1..20: mol_type = other RNA
cccatgtgttttcacactct

SEQ ID NO: 3549 - RNA, 20 nt, synthetic construct
  source 1..20: mol_type = other RNA
ggggcattacattagaaacc

SEQ ID NO: 3550 - RNA, 20 nt, synthetic construct
  source 1..20: mol_type = other RNA
gggcattacattagaaacct

SEQ ID NO: 3551 - RNA, 20 nt, synthetic construct
  source 1..20: mol_type = other RNA
gatattaattgacaggtccc

SEQ ID NO: 3552 - RNA, 20 nt, synthetic construct
  source 1..20: mol_type = other RNA
ggaaaatgatattaattgac

SEQ ID NO: 3553 - RNA, 20 nt, synthetic construct
  source 1..20: mol_type = other RNA
atgtattttcttcatgttgg

SEQ ID NO: 3554 - RNA, 20 nt, synthetic construct
  source 1..20: mol_type = other RNA
tggatgtattttcttcatgt

SEQ ID NO: 3555 - RNA, 20 nt, synthetic construct
  source 1..20: mol_type = other RNA
gagctcagtcttctcattta

SEQ ID NO: 3556 - RNA, 20 nt, synthetic construct
  source 1..20: mol_type = other RNA
taaatgagaagactgagctc

SEQ ID NO: 3557 - RNA, 20 nt, synthetic construct
  source 1..20: mol_type = other RNA
cagtcttctcatttatggaa

SEQ ID NO: 3558 - RNA, 20 nt, synthetic construct
  source 1..20: mol_type = other RNA
agtcttctcatttatggaat

SEQ ID NO: 3559 - RNA, 20 nt, synthetic construct
  source 1..20: mol_type = other RNA
gtcttctcatttatggaatg

SEQ ID NO: 3560 - RNA, 20 nt, synthetic construct
  source 1..20: mol_type = other RNA
tcatagttgtcttttagacc

SEQ ID NO: 3561 - RNA, 20 nt, synthetic construct
  source 1..20: mol_type = other RNA
gtctaaaagacaactatgaa

SEQ ID NO: 3562 - RNA, 20 nt, synthetic construct
  source 1..20: mol_type = other RNA
ttcttatacattatctttcc

SEQ ID NO: 3563 - RNA, 20 nt, synthetic construct
  source 1..20: mol_type = other RNA
acctagaatcatctttgaca

SEQ ID NO: 3564 - RNA, 20 nt, synthetic construct
  source 1..20: mol_type = other RNA
cctagaatcatctttgacat

SEQ ID NO: 3565 - RNA, 20 nt, synthetic construct
  source 1..20: mol_type = other RNA
ctagaatcatctttgacatg

SEQ ID NO: 3566 - RNA, 20 nt, synthetic construct
  source 1..20: mol_type = other RNA
gaatcatctttgacatgggg

SEQ ID NO: 3567 - RNA, 20 nt, synthetic construct
  source 1..20: mol_type = other RNA
aatcatctttgacatggggt

SEQ ID NO: 3568 - RNA, 20 nt, synthetic construct
  source 1..20: mol_type = other RNA
gggatatgtctcatcataat

SEQ ID NO: 3569 - RNA, 20 nt, synthetic construct
  source 1..20: mol_type = other RNA
ctcaaagggactctttttca

SEQ ID NO: 3570 - RNA, 20 nt, synthetic construct
  source 1..20: mol_type = other RNA
actcaaagggactctttttc

SEQ ID NO: 3571 - RNA, 20 nt, synthetic construct
  source 1..20: mol_type = other RNA
tttgagtgtcttcgtctttc

SEQ ID NO: 3572 - RNA, 20 nt, synthetic construct
  source 1..20: mol_type = other RNA
gaaagacgaagacactcaaa

SEQ ID NO: 3573 - RNA, 20 nt, synthetic construct
  source 1..20: mol_type = other RNA
ggaaagacgaagacactcaa

SEQ ID NO: 3574 - RNA, 20 nt, synthetic construct
  source 1..20: mol_type = other RNA
gaatcagcagatgattcagc

SEQ ID NO: 3575 - RNA, 20 nt, synthetic construct
  source 1..20: mol_type = other RNA
tcatctgctgattcaagaag

SEQ ID NO: 3576 - RNA, 20 nt, synthetic construct
  source 1..20: mol_type = other RNA
tctgctgattcaagaagagg

SEQ ID NO: 3577 - RNA, 20 nt, synthetic construct
  source 1..20: mol_type = other RNA
gccatatgcagacagcacaa

SEQ ID NO: 3578 - RNA, 20 nt, synthetic construct
  source 1..20: mol_type = other RNA
ccatatgcagacagcacaaa

SEQ ID NO: 3579 - RNA, 20 nt, synthetic construct
  source 1..20: mol_type = other RNA
ccctttgtgctgtctgcata

SEQ ID NO: 3580 - RNA, 20 nt, synthetic construct
  source 1..20: mol_type = other RNA
gcacaaagggaactccccca

SEQ ID NO: 3581 - RNA, 20 nt, synthetic construct
  source 1..20: mol_type = other RNA
ctcccccatggagcttcaga

SEQ ID NO: 3582 - RNA, 20 nt, synthetic construct
  source 1..20: mol_type = other RNA
taccatctgaagctccatgg

SEQ ID NO: 3583 - RNA, 20 nt, synthetic construct
  source 1..20: mol_type = other RNA
ctaccatctgaagctccatg

SEQ ID NO: 3584 - RNA, 20 nt, synthetic construct
  source 1..20: mol_type = other RNA
gctaccatctgaagctccat

SEQ ID NO: 3585 - RNA, 20 nt, synthetic construct
  source 1..20: mol_type = other RNA
ggctaccatctgaagctcca

SEQ ID NO: 3586 - RNA, 20 nt, synthetic construct
  source 1..20: mol_type = other RNA
tgaataattaagtgagtgca

SEQ ID NO: 3587 - RNA, 20 nt, synthetic construct
  source 1..20: mol_type = other RNA
gtgaataattaagtgagtgc

SEQ ID NO: 3588 - RNA, 20 nt, synthetic construct
  source 1..20: mol_type = other RNA
atgtcaggcagatttcatgc

SEQ ID NO: 3589 - RNA, 20 nt, synthetic construct
  source 1..20: mol_type = other RNA
ggatgaggaagagggatgtc

SEQ ID NO: 3590 - RNA, 20 nt, synthetic construct
  source 1..20: mol_type = other RNA
tgtcaagaggatgaggaaga

SEQ ID NO: 3591 - RNA, 20 nt, synthetic construct
  source 1..20: mol_type = other RNA
ctgtcaagaggatgaggaag

SEQ ID NO: 3592 - RNA, 20 nt, synthetic construct
  source 1..20: mol_type = other RNA
ctgttgctgtcaagaggatg

SEQ ID NO: 3593 - RNA, 20 nt, synthetic construct
  source 1..20: mol_type = other RNA
cttgacagcaacagcattaa

SEQ ID NO: 3594 - RNA, 20 nt, synthetic construct
  source 1..20: mol_type = other RNA
ttaatgctgttgctgtcaag

SEQ ID NO: 3595 - RNA, 20 nt, synthetic construct
  source 1..20: mol_type = other RNA
ttaaaggattaagtagtatt

SEQ ID NO: 3596 - RNA, 20 nt, synthetic construct
  source 1..20: mol_type = other RNA
taaaggattaagtagtattt

SEQ ID NO: 3597 - RNA, 20 nt, synthetic construct
  source 1..20: mol_type = other RNA
aaaggattaagtagtatttg

SEQ ID NO: 3598 - RNA, 20 nt, synthetic construct
  source 1..20: mol_type = other RNA
agtagtatttggggctctga

SEQ ID NO: 3599 - RNA, 20 nt, synthetic construct
  source 1..20: mol_type = other RNA
gtagtatttggggctctgaa

SEQ ID NO: 3600 - RNA, 20 nt, synthetic construct
  source 1..20: mol_type = other RNA
tagtatttggggctctgaag

SEQ ID NO: 3601 - RNA, 20 nt, synthetic construct
  source 1..20: mol_type = other RNA
gaagagtgtttgtgtacaaa

SEQ ID NO: 3602 - RNA, 20 nt, synthetic construct
  source 1..20: mol_type = other RNA
tttgtacacaaacactcttc

SEQ ID NO: 3603 - RNA, 20 nt, synthetic construct
  source 1..20: mol_type = other RNA
aatccaagtacataagacag

SEQ ID NO: 3604 - RNA, 20 nt, synthetic construct
  source 1..20: mol_type = other RNA
tgtccgctgtcttatgtact

SEQ ID NO: 3605 - RNA, 20 nt, synthetic construct
  source 1..20: mol_type = other RNA
ataagacagcggacatcact

SEQ ID NO: 3606 - RNA, 20 nt, synthetic construct
  source 1..20: mol_type = other RNA
taagacagcggacatcactt

SEQ ID NO: 3607 - RNA, 20 nt, synthetic construct
  source 1..20: mol_type = other RNA
cattgacctcctctgtatct

SEQ ID NO: 3608 - RNA, 20 nt, synthetic construct
  source 1..20: mol_type = other RNA
cctcctctgtatctaggcaa

SEQ ID NO: 3609 - RNA, 20 nt, synthetic construct
  source 1..20: mol_type = other RNA
ccattgcctagatacagagg

SEQ ID NO: 3610 - RNA, 20 nt, synthetic construct
  source 1..20: mol_type = other RNA
agaccattgcctagatacag

SEQ ID NO: 3611 - RNA, 20 nt, synthetic construct
  source 1..20: mol_type = other RNA
atcaagcaccacacccccaa

SEQ ID NO: 3612 - RNA, 20 nt, synthetic construct
  source 1..20: mol_type = other RNA
aactgcagccattgggggtg

SEQ ID NO: 3613 - RNA, 20 nt, synthetic construct
  source 1..20: mol_type = other RNA
tggagaactgcagccattgg

SEQ ID NO: 3614 - RNA, 20 nt, synthetic construct
  source 1..20: mol_type = other RNA
atggctgcagttctccatcc

SEQ ID NO: 3615 - RNA, 20 nt, synthetic construct
  source 1..20: mol_type = other RNA
gatggagaactgcagccatt

SEQ ID NO: 3616 - RNA, 20 nt, synthetic construct
  source 1..20: mol_type = other RNA
ggatggagaactgcagccat

SEQ ID NO: 3617 - RNA, 20 nt, synthetic construct
  source 1..20: mol_type = other RNA
gcagttctccatcctggtta

SEQ ID NO: 3618 - RNA, 20 nt, synthetic construct
  source 1..20: mol_type = other RNA
aggagaggccttaaccagga

SEQ ID NO: 3619 - RNA, 20 nt, synthetic construct
  source 1..20: mol_type = other RNA
ggttaaggcctctccttctg

SEQ ID NO: 3620 - RNA, 20 nt, synthetic construct
  source 1..20: mol_type = other RNA
cagaaggagaggccttaacc

SEQ ID NO: 3621 - RNA, 20 nt, synthetic construct
  source 1..20: mol_type = other RNA
aagtcattcctcagaaggag

SEQ ID NO: 3622 - RNA, 20 nt, synthetic construct
  source 1..20: mol_type = other RNA
ggaagaagtcattcctcaga

SEQ ID NO: 3623 - RNA, 20 nt, synthetic construct
  source 1..20: mol_type = other RNA
gggttagactgactgttaaa

SEQ ID NO: 3624 - RNA, 20 nt, synthetic construct
  source 1..20: mol_type = other RNA
aacagtcagtctaaccctga

SEQ ID NO: 3625 - RNA, 20 nt, synthetic construct
  source 1..20: mol_type = other RNA
gtcagtctaaccctgagggc

SEQ ID NO: 3626 - RNA, 20 nt, synthetic construct
  source 1..20: mol_type = other RNA
tctaaccctgagggctggag

SEQ ID NO: 3627 - RNA, 20 nt, synthetic construct
  source 1..20: mol_type = other RNA
ctaaccctgagggctggaga

SEQ ID NO: 3628 - RNA, 20 nt, synthetic construct
  source 1..20: mol_type = other RNA
gtggccctctccagccctca

SEQ ID NO: 3629 - RNA, 20 nt, synthetic construct
  source 1..20: mol_type = other RNA
tgtggccctctccagccctc

SEQ ID NO: 3630 - RNA, 20 nt, synthetic construct
  source 1..20: mol_type = other RNA
ggttgtgttaatgacctctg

SEQ ID NO: 3631 - RNA, 20 nt, synthetic construct
  source 1..20: mol_type = other RNA
tctacacctgctgaacagtg

SEQ ID NO: 3632 - RNA, 20 nt, synthetic construct
  source 1..20: mol_type = other RNA
acactgttcagcaggtgtag

SEQ ID NO: 3633 - RNA, 20 nt, synthetic construct
  source 1..20: mol_type = other RNA
cacctgctgaacagtgtggc

SEQ ID NO: 3634 - RNA, 20 nt, synthetic construct
  source 1..20: mol_type = other RNA
ttcctgccacactgttcagc

SEQ ID NO: 3635 - RNA, 20 nt, synthetic construct
  source 1..20: mol_type = other RNA
cagtgtggcaggaagaacat

SEQ ID NO: 3636 - RNA, 20 nt, synthetic construct
  source 1..20: mol_type = other RNA
agtgtggcaggaagaacata

SEQ ID NO: 3637 - RNA, 20 nt, synthetic construct
  source 1..20: mol_type = other RNA
gcaggaagaacatagggctg

SEQ ID NO: 3638 - RNA, 20 nt, synthetic construct
  source 1..20: mol_type = other RNA
taataacccaagagctacct

SEQ ID NO: 3639 - RNA, 20 nt, synthetic construct
  source 1..20: mol_type = other RNA
aaggtagctcttgggttatt

SEQ ID NO: 3640 - RNA, 20 nt, synthetic construct
  source 1..20: mol_type = other RNA
cagtggccaaggtagctctt

SEQ ID NO: 3641 - RNA, 20 nt, synthetic construct
  source 1..20: mol_type = other RNA
tcagtggccaaggtagctct

SEQ ID NO: 3642 - RNA, 20 nt, synthetic construct
  source 1..20: mol_type = other RNA
taccttggccactgaccaag

SEQ ID NO: 3643 - RNA, 20 nt, synthetic construct
  source 1..20: mol_type = other RNA
accttggccactgaccaagt

SEQ ID NO: 3644 - RNA, 20 nt, synthetic construct
  source 1..20: mol_type = other RNA
ccttggccactgaccaagtg

SEQ ID NO: 3645 - RNA, 20 nt, synthetic construct
  source 1..20: mol_type = other RNA
cttggccactgaccaagtgg

SEQ ID NO: 3646 - RNA, 20 nt, synthetic construct
  source 1..20: mol_type = other RNA
ccccacttggtcagtggcca

SEQ ID NO: 3647 - RNA, 20 nt, synthetic construct
  source 1..20: mol_type = other RNA
ctgaccaagtgggggcacct

SEQ ID NO: 3648 - RNA, 20 nt, synthetic construct
  source 1..20: mol_type = other RNA
tgaccaagtgggggcacctt

SEQ ID NO: 3649 - RNA, 20 nt, synthetic construct
  source 1..20: mol_type = other RNA
aggtgcccccacttggtcag

SEQ ID NO: 3650 - RNA, 20 nt, synthetic construct
  source 1..20: mol_type = other RNA
tttcccaaggtgcccccact

SEQ ID NO: 3651 - RNA, 20 nt, synthetic construct
  source 1..20: mol_type = other RNA
cagaggatgtaactttccca

SEQ ID NO: 3652 - RNA, 20 nt, synthetic construct
  source 1..20: mol_type = other RNA
atgagaaaacagagtctcag

SEQ ID NO: 3653 - RNA, 20 nt, synthetic construct
  source 1..20: mol_type = other RNA
gactctgttttctcatccac

SEQ ID NO: 3654 - RNA, 20 nt, synthetic construct
  source 1..20: mol_type = other RNA
gttttctcatccacaggatg

SEQ ID NO: 3655 - RNA, 20 nt, synthetic construct
  source 1..20: mol_type = other RNA
aatgcaacttcctcatcctg

SEQ ID NO: 3656 - RNA, 20 nt, synthetic construct
  source 1..20: mol_type = other RNA
gatgaggaagttgcattaga

SEQ ID NO: 3657 - RNA, 20 nt, synthetic construct
  source 1..20: mol_type = other RNA
attttctgtgtcatcttgct

SEQ ID NO: 3658 - RNA, 20 nt, synthetic construct
  source 1..20: mol_type = other RNA
ttttctgtgtcatcttgctt

SEQ ID NO: 3659 - RNA, 20 nt, synthetic construct
  source 1..20: mol_type = other RNA
gtgtcatcttgcttgggcca

SEQ ID NO: 3660 - RNA, 20 nt, synthetic construct
  source 1..20: mol_type = other RNA
tgtcatcttgcttgggccat

SEQ ID NO: 3661 - RNA, 20 nt, synthetic construct
  source 1..20: mol_type = other RNA
gtcatcttgcttgggccatg

SEQ ID NO: 3662 - RNA, 20 nt, synthetic construct
  source 1..20: mol_type = other RNA
actaaatgtgtggcacccca

SEQ ID NO: 3663 - RNA, 20 nt, synthetic construct
  source 1..20: mol_type = other RNA
catttagtcaaacattattc

SEQ ID NO: 3664 - RNA, 20 nt, synthetic construct
  source 1..20: mol_type = other RNA
aacattattctggctgtttc

SEQ ID NO: 3665 - RNA, 20 nt, synthetic construct
  source 1..20: mol_type = other RNA
catttcaatctgagtaaagc

SEQ ID NO: 3666 - RNA, 20 nt, synthetic construct
  source 1..20: mol_type = other RNA
gcaggttgccctccctaaca

SEQ ID NO: 3667 - RNA, 20 nt, synthetic construct
  source 1..20: mol_type = other RNA
caggttgccctccctaacat

SEQ ID NO: 3668 - RNA, 20 nt, synthetic construct
  source 1..20: mol_type = other RNA
ttgccctccctaacatgggt

SEQ ID NO: 3669 - RNA, 20 nt, synthetic construct
  source 1..20: mol_type = other RNA
gggcctacccatgttaggga

SEQ ID NO: 3670 - RNA, 20 nt, synthetic construct
  source 1..20: mol_type = other RNA
ggggcctacccatgttaggg

SEQ ID NO: 3671 - RNA, 20 nt, synthetic construct
  source 1..20: mol_type = other RNA
tctggggcctacccatgtta

SEQ ID NO: 3672 - RNA, 20 nt, synthetic construct
  source 1..20: mol_type = other RNA
gtctggggcctacccatgtt

SEQ ID NO: 3673 - RNA, 20 nt, synthetic construct
  source 1..20: mol_type = other RNA
atgggtaggccccagacaat

SEQ ID NO: 3674 - RNA, 20 nt, synthetic construct
  source 1..20: mol_type = other RNA
ggctttcagccaattgtctg

SEQ ID NO: 3675 - RNA, 20 nt, synthetic construct
  source 1..20: mol_type = other RNA
tggctttcagccaattgtct

SEQ ID NO: 3676 - RNA, 20 nt, synthetic construct
  source 1..20: mol_type = other RNA
ctggctttcagccaattgtc

SEQ ID NO: 3677 - RNA, 20 nt, synthetic construct
  source 1..20: mol_type = other RNA
aaagccagaacagaatcaaa

SEQ ID NO: 3678 - RNA, 20 nt, synthetic construct
  source 1..20: mol_type = other RNA
tctgccttttgattctgttc

SEQ ID NO: 3679 - RNA, 20 nt, synthetic construct
  source 1..20: mol_type = other RNA
gcagacccctcctagatata

SEQ ID NO: 3680 - RNA, 20 nt, synthetic construct
  source 1..20: mol_type = other RNA
cagacccctcctagatataa

SEQ ID NO: 3681 - RNA, 20 nt, synthetic construct
  source 1..20: mol_type = other RNA
agacccctcctagatataag

SEQ ID NO: 3682 - RNA, 20 nt, synthetic construct
  source 1..20: mol_type = other RNA
gacccctcctagatataagg

SEQ ID NO: 3683 - RNA, 20 nt, synthetic construct
  source 1..20: mol_type = other RNA
ttcccccttatatctaggag

SEQ ID NO: 3684 - RNA, 20 nt, synthetic construct
  source 1..20: mol_type = other RNA
attcccccttatatctagga

SEQ ID NO: 3685 - RNA, 20 nt, synthetic construct
  source 1..20: mol_type = other RNA
gattcccccttatatctagg

SEQ ID NO: 3686 - RNA, 20 nt, synthetic construct
  source 1..20: mol_type = other RNA
agagattcccccttatatct

SEQ ID NO: 3687 - RNA, 20 nt, synthetic construct
  source 1..20: mol_type = other RNA
aaactgatgtcgcaggctca

SEQ ID NO: 3688 - RNA, 20 nt, synthetic construct
  source 1..20: mol_type = other RNA
cagggaaaaactgatgtcgc

SEQ ID NO: 3689 - RNA, 20 nt, synthetic construct
  source 1..20: mol_type = other RNA
catcagtttttccctgcctt

SEQ ID NO: 3690 - RNA, 20 nt, synthetic construct
  source 1..20: mol_type = other RNA
tcattttgagtccaaaggca

SEQ ID NO: 3691 - RNA, 20 nt, synthetic construct
  source 1..20: mol_type = other RNA
ttcattttgagtccaaaggc

SEQ ID NO: 3692 - RNA, 20 nt, synthetic construct
  source 1..20: mol_type = other RNA
ttggactcaaaatgaaacac

SEQ ID NO: 3693 - RNA, 20 nt, synthetic construct
  source 1..20: mol_type = other RNA
tggactcaaaatgaaacact

SEQ ID NO: 3694 - RNA, 20 nt, synthetic construct
  source 1..20: mol_type = other RNA
gtgtttcattttgagtccaa

SEQ ID NO: 3695 - RNA, 20 nt, synthetic construct
  source 1..20: mol_type = other RNA
atgaaacactgggttttcct

SEQ ID NO: 3696 - RNA, 20 nt, synthetic construct
  source 1..20: mol_type = other RNA
ggctggcagacttaagacct

SEQ ID NO: 3697 - RNA, 20 nt, synthetic construct
  source 1..20: mol_type = other RNA
aagtctgccagcctttgaac

SEQ ID NO: 3698 - RNA, 20 nt, synthetic construct
  source 1..20: mol_type = other RNA
gtgagttccagttcaaaggc

SEQ ID NO: 3699 - RNA, 20 nt, synthetic construct
  source 1..20: mol_type = other RNA
tgaactggaactcacaccac

SEQ ID NO: 3700 - RNA, 20 nt, synthetic construct
  source 1..20: mol_type = other RNA
tggtgtgagttccagttcaa

SEQ ID NO: 3701 - RNA, 20 nt, synthetic construct
  source 1..20: mol_type = other RNA
tggagatgcaggagagccag

SEQ ID NO: 3702 - RNA, 20 nt, synthetic construct
  source 1..20: mol_type = other RNA
actcagcatgctggagatgc

SEQ ID NO: 3703 - RNA, 20 nt, synthetic construct
  source 1..20: mol_type = other RNA
tgcagaatgactcagcatgc

SEQ ID NO: 3704 - RNA, 20 nt, synthetic construct
  source 1..20: mol_type = other RNA
ctgagtcattctgcagatct

SEQ ID NO: 3705 - RNA, 20 nt, synthetic construct
  source 1..20: mol_type = other RNA
attggcttatgtgattatgg

SEQ ID NO: 3706 - RNA, 20 nt, synthetic construct
  source 1..20: mol_type = other RNA
ggaattggcttatgtgatta

SEQ ID NO: 3707 - RNA, 20 nt, synthetic construct
  source 1..20: mol_type = other RNA
taagccaattccttatccta

SEQ ID NO: 3708 - RNA, 20 nt, synthetic construct
  source 1..20: mol_type = other RNA
aaatccttaggataaggaat

SEQ ID NO: 3709 - RNA, 20 nt, synthetic construct
  source 1..20: mol_type = other RNA
acacgtaaatccttaggata

SEQ ID NO: 3710 - RNA, 20 nt, synthetic construct
  source 1..20: mol_type = other RNA
aacaatacacgtaaatcctt

SEQ ID NO: 3711 - RNA, 20 nt, synthetic construct
  source 1..20: mol_type = other RNA
ttgttttccatccatcctat

SEQ ID NO: 3712 - RNA, 20 nt, synthetic construct
  source 1..20: mol_type = other RNA
aatagaaccaataggatgga

SEQ ID NO: 3713 - RNA, 20 nt, synthetic construct
  source 1..20: mol_type = other RNA
tcctattggttctatttccc

SEQ ID NO: 3714 - RNA, 20 nt, synthetic construct
  source 1..20: mol_type = other RNA
gggaaatagaaccaatagga

SEQ ID NO: 3715 - RNA, 20 nt, synthetic construct
  source 1..20: mol_type = other RNA
tccagggaaatagaaccaat

SEQ ID NO: 3716 - RNA, 20 nt, synthetic construct
  source 1..20: mol_type = other RNA
gattgtattaggattttcca

SEQ ID NO: 3717 - RNA, 20 nt, synthetic construct
  source 1..20: mol_type = other RNA
ggattgtattaggattttcc

SEQ ID NO: 3718 - RNA, 20 nt, synthetic construct
  source 1..20: mol_type = other RNA
tcatctttggggattgtatt

SEQ ID NO: 3719 - RNA, 20 nt, synthetic construct
  source 1..20: mol_type = other RNA
gaaatgaaagttcatctttg

SEQ ID NO: 3720 - RNA, 20 nt, synthetic construct
  source 1..20: mol_type = other RNA
agaaatgaaagttcatcttt

SEQ ID NO: 3721 - RNA, 20 nt, synthetic construct
  source 1..20: mol_type = other RNA
tagaaatgaaagttcatctt

SEQ ID NO: 3722 - RNA, 20 nt, synthetic construct
  source 1..20: mol_type = other RNA
catttctaacccctaccaaa

SEQ ID NO: 3723 - RNA, 20 nt, synthetic construct
  source 1..20: mol_type = other RNA
atcagatggccatttggtag

SEQ ID NO: 3724 - RNA, 20 nt, synthetic construct
  source 1..20: mol_type = other RNA
gatcagatggccatttggta

SEQ ID NO: 3725 - RNA, 20 nt, synthetic construct
  source 1..20: mol_type = other RNA
ggatcagatggccatttggt

SEQ ID NO: 3726 - RNA, 20 nt, synthetic construct
  source 1..20: mol_type = other RNA
aagtggatcagatggccatt

SEQ ID NO: 3727 - RNA, 20 nt, synthetic construct
  source 1..20: mol_type = other RNA
aggtgtacaagtggatcaga

SEQ ID NO: 3728 - RNA, 20 nt, synthetic construct
  source 1..20: mol_type = other RNA
gtctctaagaggtgtacaag

SEQ ID NO: 3729 - RNA, 20 nt, synthetic construct
  source 1..20: mol_type = other RNA
agtgcagtcttgtctctaag

SEQ ID NO: 3730 - RNA, 20 nt, synthetic construct
  source 1..20: mol_type = other RNA
caagactgcactgctccctg

SEQ ID NO: 3731 - RNA, 20 nt, synthetic construct
  source 1..20: mol_type = other RNA
tggcacctcaccctgctcta

SEQ ID NO: 3732 - RNA, 20 nt, synthetic construct
  source 1..20: mol_type = other RNA
agagcagggtgaggtgccac

SEQ ID NO: 3733 - RNA, 20 nt, synthetic construct
  source 1..20: mol_type = other RNA
tcaccctgctctaagggcag

SEQ ID NO: 3734 - RNA, 20 nt, synthetic construct
  source 1..20: mol_type = other RNA
ccctgctctaagggcagtgg

SEQ ID NO: 3735 - RNA, 20 nt, synthetic construct
  source 1..20: mol_type = other RNA
cctccactgcccttagagca

SEQ ID NO: 3736 - RNA, 20 nt, synthetic construct
  source 1..20: mol_type = other RNA
acctccactgcccttagagc

SEQ ID NO: 3737 - RNA, 20 nt, synthetic construct
  source 1..20: mol_type = other RNA
ggcagtggaggtcagcctct

SEQ ID NO: 3738 - RNA, 20 nt, synthetic construct
  source 1..20: mol_type = other RNA
gcagtggaggtcagcctctt

SEQ ID NO: 3739 - RNA, 20 nt, synthetic construct
  source 1..20: mol_type = other RNA
ctcttgggaagcactacccc

SEQ ID NO: 3740 - RNA, 20 nt, synthetic construct
  source 1..20: mol_type = other RNA
ctggggtagtgcttcccaag

SEQ ID NO: 3741 - RNA, 20 nt, synthetic construct
  source 1..20: mol_type = other RNA
ttcagctttggagtcacctg

SEQ ID NO: 3742 - RNA, 20 nt, synthetic construct
  source 1..20: mol_type = other RNA
gttcagctttggagtcacct

SEQ ID NO: 3743 - RNA, 20 nt, synthetic construct
  source 1..20: mol_type = other RNA
ggttcagctttggagtcacc

SEQ ID NO: 3744 - RNA, 20 nt, synthetic construct
  source 1..20: mol_type = other RNA
gaatgtggctggttcagctt

SEQ ID NO: 3745 - RNA, 20 nt, synthetic construct
  source 1..20: mol_type = other RNA
tttgtgggtgggaatgtggc

SEQ ID NO: 3746 - RNA, 20 nt, synthetic construct
  source 1..20: mol_type = other RNA
actctttgtgggtgggaatg

SEQ ID NO: 3747 - RNA, 20 nt, synthetic construct
  source 1..20: mol_type = other RNA
gagaaacactctttgtgggt

SEQ ID NO: 3748 - RNA, 20 nt, synthetic construct
  source 1..20: mol_type = other RNA
ggagaaacactctttgtggg

SEQ ID NO: 3749 - RNA, 20 nt, synthetic construct
  source 1..20: mol_type = other RNA
acaaagagtgtttctccaac

SEQ ID NO: 3750 - RNA, 20 nt, synthetic construct
  source 1..20: mol_type = other RNA
gttggagaaacactctttgt

SEQ ID NO: 3751 - RNA, 20 nt, synthetic construct
  source 1..20: mol_type = other RNA
tgttggagaaacactctttg

SEQ ID NO: 3752 - RNA, 20 nt, synthetic construct
  source 1..20: mol_type = other RNA
tcaggtcaaatcacacctgt

SEQ ID NO: 3753 - RNA, 20 nt, synthetic construct
  source 1..20: mol_type = other RNA
aatttctactgtatctgctc

SEQ ID NO: 3754 - RNA, 20 nt, synthetic construct
  source 1..20: mol_type = other RNA
acataattacagtgaaagca

SEQ ID NO: 3755 - RNA, 20 nt, synthetic construct
  source 1..20: mol_type = other RNA
gacataattacagtgaaagc

SEQ ID NO: 3756 - RNA, 20 nt, synthetic construct
  source 1..20: mol_type = other RNA
cactgtaattatgtcaatgt

SEQ ID NO: 3757 - RNA, 20 nt, synthetic construct
  source 1..20: mol_type = other RNA
aatgtaggctgagattgcct

SEQ ID NO: 3758 - RNA, 20 nt, synthetic construct
  source 1..20: mol_type = other RNA
attgccttggttgttattgt

SEQ ID NO: 3759 - RNA, 20 nt, synthetic construct
  source 1..20: mol_type = other RNA
ttgccttggttgttattgtt

SEQ ID NO: 3760 - RNA, 20 nt, synthetic construct
  source 1..20: mol_type = other RNA
aaacccaacaataacaacca

SEQ ID NO: 3761 - RNA, 20 nt, synthetic construct
  source 1..20: mol_type = other RNA
tgttgggttttatctcgttt

SEQ ID NO: 3762 - RNA, 20 nt, synthetic construct
  source 1..20: mol_type = other RNA
gttgggttttatctcgtttt

SEQ ID NO: 3763 - RNA, 20 nt, synthetic construct
  source 1..20: mol_type = other RNA
ttatctcgttttgggtttcc

SEQ ID NO: 3764 - RNA, 20 nt, synthetic construct
  source 1..20: mol_type = other RNA
ggttatcacatactgttcgt

SEQ ID NO: 3765 - RNA, 20 nt, synthetic construct
  source 1..20: mol_type = other RNA
acgaacagtatgtgataacc

SEQ ID NO: 3766 - RNA, 20 nt, synthetic construct
  source 1..20: mol_type = other RNA
tggatgtgaaaatgagttaa

SEQ ID NO: 3767 - RNA, 20 nt, synthetic construct
  source 1..20: mol_type = other RNA
atggatgtgaaaatgagtta

SEQ ID NO: 3768 - RNA, 20 nt, synthetic construct
  source 1..20: mol_type = other RNA
cattttcacatccatttcac

SEQ ID NO: 3769 - RNA, 20 nt, synthetic construct
  source 1..20: mol_type = other RNA
attttcacatccatttcact

SEQ ID NO: 3770 - RNA, 20 nt, synthetic construct
  source 1..20: mol_type = other RNA
cacatccatttcactgggtg

SEQ ID NO: 3771 - RNA, 20 nt, synthetic construct
  source 1..20: mol_type = other RNA
tttggccacacccagtgaaa

SEQ ID NO: 3772 - RNA, 20 nt, synthetic construct
  source 1..20: mol_type = other RNA
agaagtgtcaggtggtgatt

SEQ ID NO: 3773 - RNA, 20 nt, synthetic construct
  source 1..20: mol_type = other RNA
tctctttcagaagtgtcagg

SEQ ID NO: 3774 - RNA, 20 nt, synthetic construct
  source 1..20: mol_type = other RNA
aagtctctttcagaagtgtc

SEQ ID NO: 3775 - RNA, 20 nt, synthetic construct
  source 1..20: mol_type = other RNA
gaaagagacttttagtacat

SEQ ID NO: 3776 - RNA, 20 nt, synthetic construct
  source 1..20: mol_type = other RNA
aaagagacttttagtacata

SEQ ID NO: 3777 - RNA, 20 nt, synthetic construct
  source 1..20: mol_type = other RNA
agacttttagtacataggga

SEQ ID NO: 3778 - RNA, 20 nt, synthetic construct
  source 1..20: mol_type = other RNA
tggtatagtaaaaaatataa

SEQ ID NO: 3779 - RNA, 20 nt, synthetic construct
  source 1..20: mol_type = other RNA
caacatcatcttgttacctt

SEQ ID NO: 3780 - RNA, 20 nt, synthetic construct
  source 1..20: mol_type = other RNA
aacatcatcttgttacctta

SEQ ID NO: 3781 - RNA, 20 nt, synthetic construct
  source 1..20: mol_type = other RNA
ctaaggtaacaagatgatgt

SEQ ID NO: 3782 - RNA, 20 nt, synthetic construct
  source 1..20: mol_type = other RNA
ctgcaaaaattctggcccta

SEQ ID NO: 3783 - RNA, 20 nt, synthetic construct
  source 1..20: mol_type = other RNA
ggtaagaactgcaaaaattc

SEQ ID NO: 3784 - RNA, 20 nt, synthetic construct
  source 1..20: mol_type = other RNA
acatggttctttagatgaca

SEQ ID NO: 3785 - RNA, 20 nt, synthetic construct
  source 1..20: mol_type = other RNA
gacatggttctttagatgac

SEQ ID NO: 3786 - RNA, 20 nt, synthetic construct
  source 1..20: mol_type = other RNA
cacagagggagaggtggaca

SEQ ID NO: 3787 - RNA, 20 nt, synthetic construct
  source 1..20: mol_type = other RNA
ggatgacacagagggagagg

SEQ ID NO: 3788 - RNA, 20 nt, synthetic construct
  source 1..20: mol_type = other RNA
tctggatgacacagagggag

SEQ ID NO: 3789 - RNA, 20 nt, synthetic construct
  source 1..20: mol_type = other RNA
cctctgtgtcatccagagat

SEQ ID NO: 3790 - RNA, 20 nt, synthetic construct
  source 1..20: mol_type = other RNA
caatctctggatgacacaga

SEQ ID NO: 3791 - RNA, 20 nt, synthetic construct
  source 1..20: mol_type = other RNA
ccaatctctggatgacacag

SEQ ID NO: 3792 - RNA, 20 nt, synthetic construct
  source 1..20: mol_type = other RNA
gtactgtgcaatccaatctc

SEQ ID NO: 3793 - RNA, 20 nt, synthetic construct
  source 1..20: mol_type = other RNA
agtacatcattaaccctcat

SEQ ID NO: 3794 - RNA, 20 nt, synthetic construct
  source 1..20: mol_type = other RNA
cattaaccctcataggaaac

SEQ ID NO: 3795 - RNA, 20 nt, synthetic construct
  source 1..20: mol_type = other RNA
ccctcataggaaacaggaga

SEQ ID NO: 3796 - RNA, 20 nt, synthetic construct
  source 1..20: mol_type = other RNA
ccatctcctgtttcctatga

SEQ ID NO: 3797 - RNA, 20 nt, synthetic construct
  source 1..20: mol_type = other RNA
gccatctcctgtttcctatg

SEQ ID NO: 3798 - RNA, 20 nt, synthetic construct
  source 1..20: mol_type = other RNA
gctagtggggagtgcagcaa

SEQ ID NO: 3799 - RNA, 20 nt, synthetic construct
  source 1..20: mol_type = other RNA
tgctagtggggagtgcagca

SEQ ID NO: 3800 - RNA, 20 nt, synthetic construct
  source 1..20: mol_type = other RNA
cccactagcaccctccctcc

SEQ ID NO: 3801 - RNA, 20 nt, synthetic construct
  source 1..20: mol_type = other RNA
caggagggagggtgctagtg

SEQ ID NO: 3802 - RNA, 20 nt, synthetic construct
  source 1..20: mol_type = other RNA
ccaggagggagggtgctagt

SEQ ID NO: 3803 - RNA, 20 nt, synthetic construct
  source 1..20: mol_type = other RNA
gccaggagggagggtgctag

SEQ ID NO: 3804 - RNA, 20 nt, synthetic construct
  source 1..20: mol_type = other RNA
gcaccctccctcctggccag

SEQ ID NO: 3805 - RNA, 20 nt, synthetic construct
  source 1..20: mol_type = other RNA
agaccactggccaggaggga

SEQ ID NO: 3806 - RNA, 20 nt, synthetic construct
  source 1..20: mol_type = other RNA
gagaccactggccaggaggg

SEQ ID NO: 3807 - RNA, 20 nt, synthetic construct
  source 1..20: mol_type = other RNA
ctggagaccactggccagga

SEQ ID NO: 3808 - RNA, 20 nt, synthetic construct
  source 1..20: mol_type = other RNA
gctggagaccactggccagg

SEQ ID NO: 3809 - RNA, 20 nt, synthetic construct
  source 1..20: mol_type = other RNA
agagctggagaccactggcc

SEQ ID NO: 3810 - RNA, 20 nt, synthetic construct
  source 1..20: mol_type = other RNA
aagtcagagctggagaccac

SEQ ID NO: 3811 - RNA, 20 nt, synthetic construct
  source 1..20: mol_type = other RNA
ttgtaatgtgaagtcagagc

SEQ ID NO: 3812 - RNA, 20 nt, synthetic construct
  source 1..20: mol_type = other RNA
tttttttttttaagatttct

SEQ ID NO: 3813 - RNA, 20 nt, synthetic construct
  source 1..20: mol_type = other RNA
agaaaagaaagaaaaatgcc

SEQ ID NO: 3814 - RNA, 20 nt, synthetic construct
  source 1..20: mol_type = other RNA
tcagaatcagaggttgagcc

SEQ ID NO: 3815 - RNA, 20 nt, synthetic construct
  source 1..20: mol_type = other RNA
acctctgattctgatttagt

SEQ ID NO: 3816 - RNA, 20 nt, synthetic construct
  source 1..20: mol_type = other RNA
tctgattctgatttagttgg

SEQ ID NO: 3817 - RNA, 20 nt, synthetic construct
  source 1..20: mol_type = other RNA
ctgattctgatttagttgga

SEQ ID NO: 3818 - RNA, 20 nt, synthetic construct
  source 1..20: mol_type = other RNA
tgattctgatttagttggag

SEQ ID NO: 3819 - RNA, 20 nt, synthetic construct
  source 1..20: mol_type = other RNA
tccaactaaatcagaatcag

SEQ ID NO: 3820 - RNA, 20 nt, synthetic construct
  source 1..20: mol_type = other RNA
tgatttagttggaggggctg

SEQ ID NO: 3821 - RNA, 20 nt, synthetic construct
  source 1..20: mol_type = other RNA
tttagttggaggggctgagg

SEQ ID NO: 3822 - RNA, 20 nt, synthetic construct
  source 1..20: mol_type = other RNA
ggctgaggaggaaagatgct

SEQ ID NO: 3823 - RNA, 20 nt, synthetic construct
  source 1..20: mol_type = other RNA
gctgaggaggaaagatgctt

SEQ ID NO: 3824 - RNA, 20 nt, synthetic construct
  source 1..20: mol_type = other RNA
ggcattagtaagaatgcttt

SEQ ID NO: 3825 - RNA, 20 nt, synthetic construct
  source 1..20: mol_type = other RNA
aggtgattctaatgtacagc

SEQ ID NO: 3826 - RNA, 20 nt, synthetic construct
  source 1..20: mol_type = other RNA
tgagaaccagtgttctgtct

SEQ ID NO: 3827 - RNA, 20 nt, synthetic construct
  source 1..20: mol_type = other RNA
ctctggcctagacagaacac

SEQ ID NO: 3828 - RNA, 20 nt, synthetic construct
  source 1..20: mol_type = other RNA
agacaaagtttgctgatctc

SEQ ID NO: 3829 - RNA, 20 nt, synthetic construct
  source 1..20: mol_type = other RNA
agccagaaagcaaatattat

SEQ ID NO: 3830 - RNA, 20 nt, synthetic construct
  source 1..20: mol_type = other RNA
agcctataatatttgctttc

SEQ ID NO: 3831 - RNA, 20 nt, synthetic construct
  source 1..20: mol_type = other RNA
agcaaatattataggctttg

SEQ ID NO: 3832 - RNA, 20 nt, synthetic construct
  source 1..20: mol_type = other RNA
gcaaatattataggctttgc

SEQ ID NO: 3833 - RNA, 20 nt, synthetic construct
  source 1..20: mol_type = other RNA
tataggctttgcgggccaaa

SEQ ID NO: 3834 - RNA, 20 nt, synthetic construct
  source 1..20: mol_type = other RNA
cagttgctttagagaccatt

SEQ ID NO: 3835 - RNA, 20 nt, synthetic construct
  source 1..20: mol_type = other RNA
aacaatacataataaacaaa

SEQ ID NO: 3836 - RNA, 20 nt, synthetic construct
  source 1..20: mol_type = other RNA
acaatacataataaacaaat

SEQ ID NO: 3837 - RNA, 20 nt, synthetic construct
  source 1..20: mol_type = other RNA
ttttataaataaagttgtat

SEQ ID NO: 3838 - RNA, 20 nt, synthetic construct
  source 1..20: mol_type = other RNA
tatttataaaaacaagcaac

SEQ ID NO: 3839 - RNA, 20 nt, synthetic construct
  source 1..20: mol_type = other RNA
aaatagcttctggggcaaaa

SEQ ID NO: 3840 - RNA, 20 nt, synthetic construct
  source 1..20: mol_type = other RNA
aactaatgaaatagcttctg

SEQ ID NO: 3841 - RNA, 20 nt, synthetic construct
  source 1..20: mol_type = other RNA
caactaatgaaatagcttct

SEQ ID NO: 3842 - RNA, 20 nt, synthetic construct
  source 1..20: mol_type = other RNA
tcaactaatgaaatagcttc

SEQ ID NO: 3843 - RNA, 20 nt, synthetic construct
  source 1..20: mol_type = other RNA
acccagttttaaaatagttg

SEQ ID NO: 3844 - RNA, 20 nt, synthetic construct
  source 1..20: mol_type = other RNA
cccagttttaaaatagttgt

SEQ ID NO: 3845 - RNA, 20 nt, synthetic construct
  source 1..20: mol_type = other RNA
cccacaactattttaaaact

SEQ ID NO: 3846 - RNA, 20 nt, synthetic construct
  source 1..20: mol_type = other RNA
gcccacaactattttaaaac

SEQ ID NO: 3847 - RNA, 20 nt, synthetic construct
  source 1..20: mol_type = other RNA
tagttgtgggcccagcacag

SEQ ID NO: 3848 - RNA, 20 nt, synthetic construct
  source 1..20: mol_type = other RNA
caggtgtgagccactgtgct

SEQ ID NO: 3849 - RNA, 20 nt, synthetic construct
  source 1..20: mol_type = other RNA
acaggtgtgagccactgtgc

SEQ ID NO: 3850 - RNA, 20 nt, synthetic construct
  source 1..20: mol_type = other RNA
tctgaaagctctgggattac

SEQ ID NO: 3851 - RNA, 20 nt, synthetic construct
  source 1..20: mol_type = other RNA
agagctttcagagtcggaga

SEQ ID NO: 3852 - RNA, 20 nt, synthetic construct
  source 1..20: mol_type = other RNA
tctccgactctgaaagctct

SEQ ID NO: 3853 - RNA, 20 nt, synthetic construct
  source 1..20: mol_type = other RNA
ttctccgactctgaaagctc

SEQ ID NO: 3854 - RNA, 20 nt, synthetic construct
  source 1..20: mol_type = other RNA
ctttcagagtcggagaagga

SEQ ID NO: 3855 - RNA, 20 nt, synthetic construct
  source 1..20: mol_type = other RNA
ggagaaggaaggactgcttg

SEQ ID NO: 3856 - RNA, 20 nt, synthetic construct
  source 1..20: mol_type = other RNA
aggaaggactgcttgaggcc

SEQ ID NO: 3857 - RNA, 20 nt, synthetic construct
  source 1..20: mol_type = other RNA
tgcttgaggccaggagatca

SEQ ID NO: 3858 - RNA, 20 nt, synthetic construct
  source 1..20: mol_type = other RNA
tcattgtaaccttgatctcc

SEQ ID NO: 3859 - RNA, 20 nt, synthetic construct
  source 1..20: mol_type = other RNA
tatgatcatgcactccagcc

SEQ ID NO: 3860 - RNA, 20 nt, synthetic construct
  source 1..20: mol_type = other RNA
atgatcatgcactccagcct

SEQ ID NO: 3861 - RNA, 20 nt, synthetic construct
  source 1..20: mol_type = other RNA
tcttactctgttgcccaggc

SEQ ID NO: 3862 - RNA, 20 nt, synthetic construct
  source 1..20: mol_type = other RNA
agggtcttactctgttgccc

SEQ ID NO: 3863 - RNA, 20 nt, synthetic construct
  source 1..20: mol_type = other RNA
tttttttgttctaagtgaca

SEQ ID NO: 3864 - RNA, 20 nt, synthetic construct
  source 1..20: mol_type = other RNA
ttttttttgttctaagtgac

SEQ ID NO: 3865 - RNA, 20 nt, synthetic construct
  source 1..20: mol_type = other RNA
acacacacacacacacacac

SEQ ID NO: 3866 - RNA, 20 nt, synthetic construct
  source 1..20: mol_type = other RNA
acacacacacacactggtta

SEQ ID NO: 3867 - RNA, 20 nt, synthetic construct
  source 1..20: mol_type = other RNA
ctctggtgtcacagacaaga

SEQ ID NO: 3868 - RNA, 20 nt, synthetic construct
  source 1..20: mol_type = other RNA
gacaccagagactctcaaag

SEQ ID NO: 3869 - RNA, 20 nt, synthetic construct
  source 1..20: mol_type = other RNA
ccagagactctcaaagtggc

SEQ ID NO: 3870 - RNA, 20 nt, synthetic construct
  source 1..20: mol_type = other RNA
ccagccactttgagagtctc

SEQ ID NO: 3871 - RNA, 20 nt, synthetic construct
  source 1..20: mol_type = other RNA
atcaatattcactctctatc

SEQ ID NO: 3872 - RNA, 20 nt, synthetic construct
  source 1..20: mol_type = other RNA
ctgatacatgaagggaatgc

SEQ ID NO: 3873 - RNA, 20 nt, synthetic construct
  source 1..20: mol_type = other RNA
tcattcgtctgatacatgaa

SEQ ID NO: 3874 - RNA, 20 nt, synthetic construct
  source 1..20: mol_type = other RNA
atcattcgtctgatacatga

SEQ ID NO: 3875 - RNA, 20 nt, synthetic construct
  source 1..20: mol_type = other RNA
agtctttttcttgtttagat

SEQ ID NO: 3876 - RNA, 20 nt, synthetic construct
  source 1..20: mol_type = other RNA
aagtctttttcttgtttaga

SEQ ID NO: 3877 - RNA, 20 nt, synthetic construct
  source 1..20: mol_type = other RNA
agaaaaagacttgttcttag

SEQ ID NO: 3878 - RNA, 20 nt, synthetic construct
  source 1..20: mol_type = other RNA
gtgagtaatgggagacagaa

SEQ ID NO: 3879 - RNA, 20 nt, synthetic construct
  source 1..20: mol_type = other RNA
ataaggcagcagtgagtaat

SEQ ID NO: 3880 - RNA, 20 nt, synthetic construct
  source 1..20: mol_type = other RNA
aataaggcagcagtgagtaa

SEQ ID NO: 3881 - RNA, 20 nt, synthetic construct
  source 1..20: mol_type = other RNA
acgtttgtgaacatataata

SEQ ID NO: 3882 - RNA, 20 nt, synthetic construct
  source 1..20: mol_type = other RNA
tgagcttaagtcagtttctg

SEQ ID NO: 3883 - RNA, 20 nt, synthetic construct
  source 1..20: mol_type = other RNA
atggtttggaaactacagat

SEQ ID NO: 3884 - RNA, 20 nt, synthetic construct
  source 1..20: mol_type = other RNA
catggtttggaaactacaga

SEQ ID NO: 3885 - RNA, 20 nt, synthetic construct
  source 1..20: mol_type = other RNA
tcaagggggaaagcatggtt

SEQ ID NO: 3886 - RNA, 20 nt, synthetic construct
  source 1..20: mol_type = other RNA
atgctttcccccttgaaagc

SEQ ID NO: 3887 - RNA, 20 nt, synthetic construct
  source 1..20: mol_type = other RNA
tgctttcccccttgaaagct

SEQ ID NO: 3888 - RNA, 20 nt, synthetic construct
  source 1..20: mol_type = other RNA
agctttcaagggggaaagca

SEQ ID NO: 3889 - RNA, 20 nt, synthetic construct
  source 1..20: mol_type = other RNA
acatgtcccagctttcaagg

SEQ ID NO: 3890 - RNA, 20 nt, synthetic construct
  source 1..20: mol_type = other RNA
aacatgtcccagctttcaag

SEQ ID NO: 3891 - RNA, 20 nt, synthetic construct
  source 1..20: mol_type = other RNA
aaacatgtcccagctttcaa

SEQ ID NO: 3892 - RNA, 20 nt, synthetic construct
  source 1..20: mol_type = other RNA
caaacatgtcccagctttca

SEQ ID NO: 3893 - RNA, 20 nt, synthetic construct
  source 1..20: mol_type = other RNA
caaaatcatttacaatcttc

SEQ ID NO: 3894 - RNA, 20 nt, synthetic construct
  source 1..20: mol_type = other RNA
ttttgtgaatcaaggagaat

SEQ ID NO: 3895 - RNA, 20 nt, synthetic construct
  source 1..20: mol_type = other RNA
agataatattttgtgaatca

SEQ ID NO: 3896 - RNA, 20 nt, synthetic construct
  source 1..20: mol_type = other RNA
tcacaaaatattatctaaag

SEQ ID NO: 3897 - RNA, 20 nt, synthetic construct
  source 1..20: mol_type = other RNA
ggaacttgcagatgtgattg

SEQ ID NO: 3898 - RNA, 20 nt, synthetic construct
  source 1..20: mol_type = other RNA
tgcaagttccttccgtgccc

SEQ ID NO: 3899 - RNA, 20 nt, synthetic construct
  source 1..20: mol_type = other RNA
aagttccttccgtgcccagg

SEQ ID NO: 3900 - RNA, 20 nt, synthetic construct
  source 1..20: mol_type = other RNA
tccgtgcccaggaggcgtaa

SEQ ID NO: 3901 - RNA, 20 nt, synthetic construct
  source 1..20: mol_type = other RNA
ttacgcctcctgggcacgga

SEQ ID NO: 3902 - RNA, 20 nt, synthetic construct
  source 1..20: mol_type = other RNA
gcctttacgcctcctgggca

SEQ ID NO: 3903 - RNA, 20 nt, synthetic construct
  source 1..20: mol_type = other RNA
aaaatgcctttacgcctcct

SEQ ID NO: 3904 - RNA, 20 nt, synthetic construct
  source 1..20: mol_type = other RNA
aaaaatgcctttacgcctcc

SEQ ID NO: 3905 - RNA, 20 nt, synthetic construct
  source 1..20: mol_type = other RNA
tctcattatctcttctatct

SEQ ID NO: 3906 - RNA, 20 nt, synthetic construct
  source 1..20: mol_type = other RNA
ctcattatctcttctatctt

SEQ ID NO: 3907 - RNA, 20 nt, synthetic construct
  source 1..20: mol_type = other RNA
agggtagaataaacatggtt

SEQ ID NO: 3908 - RNA, 20 nt, synthetic construct
  source 1..20: mol_type = other RNA
tggaaagggtagaataaaca

SEQ ID NO: 3909 - RNA, 20 nt, synthetic construct
  source 1..20: mol_type = other RNA
aatgatctttaagttggaaa

SEQ ID NO: 3910 - RNA, 20 nt, synthetic construct
  source 1..20: mol_type = other RNA
aaatgatctttaagttggaa

SEQ ID NO: 3911 - RNA, 20 nt, synthetic construct
  source 1..20: mol_type = other RNA
aggaaaaatgatctttaagt

SEQ ID NO: 3912 - RNA, 20 nt, synthetic construct
  source 1..20: mol_type = other RNA
ttgattttatcatctttatc

SEQ ID NO: 3913 - RNA, 20 nt, synthetic construct
  source 1..20: mol_type = other RNA
tatagagtaaacaaatgaca

SEQ ID NO: 3914 - RNA, 20 nt, synthetic construct
  source 1..20: mol_type = other RNA
tataccatctgttctaaata

SEQ ID NO: 3915 - RNA, 20 nt, synthetic construct
  source 1..20: mol_type = other RNA
atagccttatttagaacaga

SEQ ID NO: 3916 - RNA, 20 nt, synthetic construct
  source 1..20: mol_type = other RNA
taaggctatgtccttttttg

SEQ ID NO: 3917 - RNA, 20 nt, synthetic construct
  source 1..20: mol_type = other RNA
aaggctatgtccttttttgt

SEQ ID NO: 3918 - RNA, 20 nt, synthetic construct
  source 1..20: mol_type = other RNA
aggctatgtccttttttgtg

SEQ ID NO: 3919 - RNA, 20 nt, synthetic construct
  source 1..20: mol_type = other RNA
tggagcactccccacaaaaa

SEQ ID NO: 3920 - RNA, 20 nt, synthetic construct
  source 1..20: mol_type = other RNA
agttttaaaacaatactatt

SEQ ID NO: 3921 - RNA, 20 nt, synthetic construct
  source 1..20: mol_type = other RNA
gttttaaaactcttatatac

SEQ ID NO: 3922 - RNA, 20 nt, synthetic construct
  source 1..20: mol_type = other RNA
atacaggcaaccacactttc

SEQ ID NO: 3923 - RNA, 20 nt, synthetic construct
  source 1..20: mol_type = other RNA
cacactttctggttcacctc

SEQ ID NO: 3924 - RNA, 20 nt, synthetic construct
  source 1..20: mol_type = other RNA
ctgaggtgaaccagaaagtg

SEQ ID NO: 3925 - RNA, 20 nt, synthetic construct
  source 1..20: mol_type = other RNA
ctggttcacctcaggcactc

SEQ ID NO: 3926 - RNA, 20 nt, synthetic construct
  source 1..20: mol_type = other RNA
agtatataccagagtgcctg

SEQ ID NO: 3927 - RNA, 20 nt, synthetic construct
  source 1..20: mol_type = other RNA
ctggtatatactgtctgccc

SEQ ID NO: 3928 - RNA, 20 nt, synthetic construct
  source 1..20: mol_type = other RNA
tggtatatactgtctgccct

SEQ ID NO: 3929 - RNA, 20 nt, synthetic construct
  source 1..20: mol_type = other RNA
ggtatatactgtctgccctg

SEQ ID NO: 3930 - RNA, 20 nt, synthetic construct
  source 1..20: mol_type = other RNA
cctggggtaaatacgaatag

SEQ ID NO: 3931 - RNA, 20 nt, synthetic construct
  source 1..20: mol_type = other RNA
ctctattcgtatttacccca

SEQ ID NO: 3932 - RNA, 20 nt, synthetic construct
  source 1..20: mol_type = other RNA
cctctattcgtatttacccc

SEQ ID NO: 3933 - RNA, 20 nt, synthetic construct
  source 1..20: mol_type = other RNA
tctttactctgaaaagtgtc

SEQ ID NO: 3934 - RNA, 20 nt, synthetic construct
  source 1..20: mol_type = other RNA
agacacttttcagagtaaag

SEQ ID NO: 3935 - RNA, 20 nt, synthetic construct
  source 1..20: mol_type = other RNA
tgtctggttttttgaacagc

SEQ ID NO: 3936 - RNA, 20 nt, synthetic construct
  source 1..20: mol_type = other RNA
aataagtaaagctgaagaaa

SEQ ID NO: 3937 - RNA, 20 nt, synthetic construct
  source 1..20: mol_type = other RNA
gaaatggtaaagcactccac

SEQ ID NO: 3938 - RNA, 20 nt, synthetic construct
  source 1..20: mol_type = other RNA
aaatggtaaagcactccaca

SEQ ID NO: 3939 - RNA, 20 nt, synthetic construct
  source 1..20: mol_type = other RNA
aaagcactccacagggttca

SEQ ID NO: 3940 - RNA, 20 nt, synthetic construct
  source 1..20: mol_type = other RNA
aagcactccacagggttcat

SEQ ID NO: 3941 - RNA, 20 nt, synthetic construct
  source 1..20: mol_type = other RNA
cacagggttcatgggctctc

SEQ ID NO: 3942 - RNA, 20 nt, synthetic construct
  source 1..20: mol_type = other RNA
ctgagagcccatgaaccctg

SEQ ID NO: 3943 - RNA, 20 nt, synthetic construct
  source 1..20: mol_type = other RNA
ttctctttttcttgaatgtg

SEQ ID NO: 3944 - RNA, 20 nt, synthetic construct
  source 1..20: mol_type = other RNA
actatttctgttgaaaactt

SEQ ID NO: 3945 - RNA, 20 nt, synthetic construct
  source 1..20: mol_type = other RNA
gttgaaaactttggccacac

SEQ ID NO: 3946 - RNA, 20 nt, synthetic construct
  source 1..20: mol_type = other RNA
ttgaaaactttggccacact

SEQ ID NO: 3947 - RNA, 20 nt, synthetic construct
  source 1..20: mol_type = other RNA
aactttggccacactgggcc

SEQ ID NO: 3948 - RNA, 20 nt, synthetic construct
  source 1..20: mol_type = other RNA
tggccacactgggccaggca

SEQ ID NO: 3949 - RNA, 20 nt, synthetic construct
  source 1..20: mol_type = other RNA
tgaccatgcctggcccagtg

SEQ ID NO: 3950 - RNA, 20 nt, synthetic construct
  source 1..20: mol_type = other RNA
attacaggtgtgaccatgcc

SEQ ID NO: 3951 - RNA, 20 nt, synthetic construct
  source 1..20: mol_type = other RNA
cacctgtaatcccagaactt

SEQ ID NO: 3952 - RNA, 20 nt, synthetic construct
  source 1..20: mol_type = other RNA
acctgtaatcccagaacttt

SEQ ID NO: 3953 - RNA, 20 nt, synthetic construct
  source 1..20: mol_type = other RNA
tcccaaagttctgggattac

SEQ ID NO: 3954 - RNA, 20 nt, synthetic construct
  source 1..20: mol_type = other RNA
agaactttgggaagccaaga

SEQ ID NO: 3955 - RNA, 20 nt, synthetic construct
  source 1..20: mol_type = other RNA
gaactttgggaagccaagac

SEQ ID NO: 3956 - RNA, 20 nt, synthetic construct
  source 1..20: mol_type = other RNA
tcttggcttcccaaagttct

SEQ ID NO: 3957 - RNA, 20 nt, synthetic construct
  source 1..20: mol_type = other RNA
gtcttggcttcccaaagttc

SEQ ID NO: 3958 - RNA, 20 nt, synthetic construct
  source 1..20: mol_type = other RNA
ctttgggaagccaagacggg

SEQ ID NO: 3959 - RNA, 20 nt, synthetic construct
  source 1..20: mol_type = other RNA
ctcaggtgatccacccgtct

SEQ ID NO: 3960 - RNA, 20 nt, synthetic construct
  source 1..20: mol_type = other RNA
cgggtggatcacctgagatc

SEQ ID NO: 3961 - RNA, 20 nt, synthetic construct
  source 1..20: mol_type = other RNA
ggtctcgaactcctgatctc

SEQ ID NO: 3962 - RNA, 20 nt, synthetic construct
  source 1..20: mol_type = other RNA
tcaggagttcgagaccagcg

SEQ ID NO: 3963 - RNA, 20 nt, synthetic construct
  source 1..20: mol_type = other RNA
cgagaccagcgtggccaaca

SEQ ID NO: 3964 - RNA, 20 nt, synthetic construct
  source 1..20: mol_type = other RNA
tttcaccgtgttggccacgc

SEQ ID NO: 3965 - RNA, 20 nt, synthetic construct
  source 1..20: mol_type = other RNA
gagacagagtttcaccgtgt

SEQ ID NO: 3966 - RNA, 20 nt, synthetic construct
  source 1..20: mol_type = other RNA
caaaaatacaaaaattagcc

SEQ ID NO: 3967 - RNA, 20 nt, synthetic construct
  source 1..20: mol_type = other RNA
ctggctaatttttgtatttt

SEQ ID NO: 3968 - RNA, 20 nt, synthetic construct
  source 1..20: mol_type = other RNA
atacaaaaattagccaggca

SEQ ID NO: 3969 - RNA, 20 nt, synthetic construct
  source 1..20: mol_type = other RNA
caaaaattagccaggcatgg

SEQ ID NO: 3970 - RNA, 20 nt, synthetic construct
  source 1..20: mol_type = other RNA
aaattagccaggcatggtgg

SEQ ID NO: 3971 - RNA, 20 nt, synthetic construct
  source 1..20: mol_type = other RNA
aattagccaggcatggtggc

SEQ ID NO: 3972 - RNA, 20 nt, synthetic construct
  source 1..20: mol_type = other RNA
caggcgcccgccaccatgcc

SEQ ID NO: 3973 - RNA, 20 nt, synthetic construct
  source 1..20: mol_type = other RNA
gcctgtaatcccagctactc

SEQ ID NO: 3974 - RNA, 20 nt, synthetic construct
  source 1..20: mol_type = other RNA
tgtaatcccagctactcagg

SEQ ID NO: 3975 - RNA, 20 nt, synthetic construct
  source 1..20: mol_type = other RNA
tcctgagtagctgggattac

SEQ ID NO: 3976 - RNA, 20 nt, synthetic construct
  source 1..20: mol_type = other RNA
cccagctactcaggaggctg

SEQ ID NO: 3977 - RNA, 20 nt, synthetic construct
  source 1..20: mol_type = other RNA
gctactcaggaggctgaggc

SEQ ID NO: 3978 - RNA, 20 nt, synthetic construct
  source 1..20: mol_type = other RNA
cctcagcctcctgagtagct

SEQ ID NO: 3979 - RNA, 20 nt, synthetic construct
  source 1..20: mol_type = other RNA
gcctcagcctcctgagtagc

SEQ ID NO: 3980 - RNA, 20 nt, synthetic construct
  source 1..20: mol_type = other RNA
ggctgaggcaggagaatcac

SEQ ID NO: 3981 - RNA, 20 nt, synthetic construct
  source 1..20: mol_type = other RNA
gcaggagaatcactggaact

SEQ ID NO: 3982 - RNA, 20 nt, synthetic construct
  source 1..20: mol_type = other RNA
caggagaatcactggaactc

SEQ ID NO: 3983 - RNA, 20 nt, synthetic construct
  source 1..20: mol_type = other RNA
gagaatcactggaactcggg

SEQ ID NO: 3984 - RNA, 20 nt, synthetic construct
  source 1..20: mol_type = other RNA
cactggaactcgggaggcag

SEQ ID NO: 3985 - RNA, 20 nt, synthetic construct
  source 1..20: mol_type = other RNA
cacgccactgcacaccagcc

SEQ ID NO: 3986 - RNA, 20 nt, synthetic construct
  source 1..20: mol_type = other RNA
acgccactgcacaccagcct

SEQ ID NO: 3987 - RNA, 20 nt, synthetic construct
  source 1..20: mol_type = other RNA
ttgcccaggctggtgtgcag

SEQ ID NO: 3988 - RNA, 20 nt, synthetic construct
  source 1..20: mol_type = other RNA
tcttgctctgttgcccaggc

SEQ ID NO: 3989 - RNA, 20 nt, synthetic construct
  source 1..20: mol_type = other RNA
agagtcttgctctgttgccc

SEQ ID NO: 3990 - RNA, 20 nt, synthetic construct
  source 1..20: mol_type = other RNA
aaaaaaaactctagccacac

SEQ ID NO: 3991 - RNA, 20 nt, synthetic construct
  source 1..20: mol_type = other RNA
ccacactggattcatatcct

SEQ ID NO: 3992 - RNA, 20 nt, synthetic construct
  source 1..20: mol_type = other RNA
cctaggatatgaatccagtg

SEQ ID NO: 3993 - RNA, 20 nt, synthetic construct
  source 1..20: mol_type = other RNA
aactagtaagtggcaggcct

SEQ ID NO: 3994 - RNA, 20 nt, synthetic construct
  source 1..20: mol_type = other RNA
tcatagaactagtaagtggc

SEQ ID NO: 3995 - RNA, 20 nt, synthetic construct
  source 1..20: mol_type = other RNA
cttactagttctatgaccac

SEQ ID NO: 3996 - RNA, 20 nt, synthetic construct
  source 1..20: mol_type = other RNA
gtggtcatagaactagtaag

SEQ ID NO: 3997 - RNA, 20 nt, synthetic construct
  source 1..20: mol_type = other RNA
agattgggtaacttatcctg

SEQ ID NO: 3998 - RNA, 20 nt, synthetic construct
  source 1..20: mol_type = other RNA
agctgagagttaaagagatt

SEQ ID NO: 3999 - RNA, 20 nt, synthetic construct
  source 1..20: mol_type = other RNA
gagctgagagttaaagagat

SEQ ID NO: 4000 - RNA, 20 nt, synthetic construct
  source 1..20: mol_type = other RNA
taactctcagctcaactcac

SEQ ID NO: 4001 - RNA, 20 nt, synthetic construct
  source 1..20: mol_type = other RNA
tcatgcatttagtattaaat

SEQ ID NO: 4002 - RNA, 20 nt, synthetic construct
  source 1..20: mol_type = other RNA
gtaatattggcaatgataat

SEQ ID NO: 4003 - RNA, 20 nt, synthetic construct
  source 1..20: mol_type = other RNA
aataacactgatagtaatat

SEQ ID NO: 4004 - RNA, 20 nt, synthetic construct
  source 1..20: mol_type = other RNA
tcaacccctccacagcaaca

SEQ ID NO: 4005 - RNA, 20 nt, synthetic construct
  source 1..20: mol_type = other RNA
tgttgctgtggaggggttga

SEQ ID NO: 4006 - RNA, 20 nt, synthetic construct
  source 1..20: mol_type = other RNA
atgttgctgtggaggggttg

SEQ ID NO: 4007 - RNA, 20 nt, synthetic construct
  source 1..20: mol_type = other RNA
gataccatgttgctgtggag

SEQ ID NO: 4008 - RNA, 20 nt, synthetic construct
  source 1..20: mol_type = other RNA
agataccatgttgctgtgga

SEQ ID NO: 4009 - RNA, 20 nt, synthetic construct
  source 1..20: mol_type = other RNA
cagataccatgttgctgtgg

SEQ ID NO: 4010 - RNA, 20 nt, synthetic construct
  source 1..20: mol_type = other RNA
tcacagataccatgttgctg

SEQ ID NO: 4011 - RNA, 20 nt, synthetic construct
  source 1..20: mol_type = other RNA
tggtatctgtgactctctat

SEQ ID NO: 4012 - RNA, 20 nt, synthetic construct
  source 1..20: mol_type = other RNA
atgtgacattctgaaaagga

SEQ ID NO: 4013 - RNA, 20 nt, synthetic construct
  source 1..20: mol_type = other RNA
caagatgtgacattctgaaa

SEQ ID NO: 4014 - RNA, 20 nt, synthetic construct
  source 1..20: mol_type = other RNA
tctcaccaatctcttgctac

SEQ ID NO: 4015 - RNA, 20 nt, synthetic construct
  source 1..20: mol_type = other RNA
ttaaaccagtagcaagagat

SEQ ID NO: 4016 - RNA, 20 nt, synthetic construct
  source 1..20: mol_type = other RNA
gactttacgagattgtgggg

SEQ ID NO: 4017 - RNA, 20 nt, synthetic construct
  source 1..20: mol_type = other RNA
aaagactttacgagattgtg

SEQ ID NO: 4018 - RNA, 20 nt, synthetic construct
  source 1..20: mol_type = other RNA
gaaagactttacgagattgt

SEQ ID NO: 4019 - RNA, 20 nt, synthetic construct
  source 1..20: mol_type = other RNA
agaaagactttacgagattg

SEQ ID NO: 4020 - RNA, 20 nt, synthetic construct
  source 1..20: mol_type = other RNA
ctttgtcttcactagaaatc

SEQ ID NO: 4021 - RNA, 20 nt, synthetic construct
  source 1..20: mol_type = other RNA
tagaaatctggaatactcca

SEQ ID NO: 4022 - RNA, 20 nt, synthetic construct
  source 1..20: mol_type = other RNA
ctccaaggaagtttcttctc

SEQ ID NO: 4023 - RNA, 20 nt, synthetic construct
  source 1..20: mol_type = other RNA
tgccagagaagaaacttcct

SEQ ID NO: 4024 - RNA, 20 nt, synthetic construct
  source 1..20: mol_type = other RNA
attatgtttgttataaatgc

SEQ ID NO: 4025 - RNA, 20 nt, synthetic construct
  source 1..20: mol_type = other RNA
acataatttgtgagctgctc

SEQ ID NO: 4026 - RNA, 20 nt, synthetic construct
  source 1..20: mol_type = other RNA
gacagttgctgagggattca

SEQ ID NO: 4027 - RNA, 20 nt, synthetic construct
  source 1..20: mol_type = other RNA
ccctcagcaactgtctttcc

SEQ ID NO: 4028 - RNA, 20 nt, synthetic construct
  source 1..20: mol_type = other RNA
ccaggaaagacagttgctga

SEQ ID NO: 4029 - RNA, 20 nt, synthetic construct
  source 1..20: mol_type = other RNA
tccaggaaagacagttgctg

SEQ ID NO: 4030 - RNA, 20 nt, synthetic construct
  source 1..20: mol_type = other RNA
taatagtttatcttgattcc

SEQ ID NO: 4031 - RNA, 20 nt, synthetic construct
  source 1..20: mol_type = other RNA
agataaactattattcttca

SEQ ID NO: 4032 - RNA, 20 nt, synthetic construct
  source 1..20: mol_type = other RNA
attattcttcatggttccct

SEQ ID NO: 4033 - RNA, 20 nt, synthetic construct
  source 1..20: mol_type = other RNA
ttattcttcatggttccctt

SEQ ID NO: 4034 - RNA, 20 nt, synthetic construct
  source 1..20: mol_type = other RNA
ttttcagagtgtgttcccaa

SEQ ID NO: 4035 - RNA, 20 nt, synthetic construct
  source 1..20: mol_type = other RNA
ggaacacactctgaaaactt

SEQ ID NO: 4036 - RNA, 20 nt, synthetic construct
  source 1..20: mol_type = other RNA
gtcattttattttctagcta

SEQ ID NO: 4037 - RNA, 20 nt, synthetic construct
  source 1..20: mol_type = other RNA
tgtcattttattttctagct

SEQ ID NO: 4038 - RNA, 20 nt, synthetic construct
  source 1..20: mol_type = other RNA
gacattaactttctgagaaa

SEQ ID NO: 4039 - RNA, 20 nt, synthetic construct
  source 1..20: mol_type = other RNA
ctgagaaaaggactgaccca

SEQ ID NO: 4040 - RNA, 20 nt, synthetic construct
  source 1..20: mol_type = other RNA
gacccaaggcatattcaaat

SEQ ID NO: 4041 - RNA, 20 nt, synthetic construct
  source 1..20: mol_type = other RNA
acccaaggcatattcaaata

SEQ ID NO: 4042 - RNA, 20 nt, synthetic construct
  source 1..20: mol_type = other RNA
cccaaggcatattcaaatag

SEQ ID NO: 4043 - RNA, 20 nt, synthetic construct
  source 1..20: mol_type = other RNA
cccctatttgaatatgcctt

SEQ ID NO: 4044 - RNA, 20 nt, synthetic construct
  source 1..20: mol_type = other RNA
tcccctatttgaatatgcct

SEQ ID NO: 4045 - RNA, 20 nt, synthetic construct
  source 1..20: mol_type = other RNA
tcaaataggggaatcataaa

SEQ ID NO: 4046 - RNA, 20 nt, synthetic construct
  source 1..20: mol_type = other RNA
caaataggggaatcataaaa

SEQ ID NO: 4047 - RNA, 20 nt, synthetic construct
  source 1..20: mol_type = other RNA
aatcataaaagggaccacac

SEQ ID NO: 4048 - RNA, 20 nt, synthetic construct
  source 1..20: mol_type = other RNA
tcactcatttttctcctgtg

SEQ ID NO: 4049 - RNA, 20 nt, synthetic construct
  source 1..20: mol_type = other RNA
tatcttagttactcagtaaa

SEQ ID NO: 4050 - RNA, 20 nt, synthetic construct
  source 1..20: mol_type = other RNA
aactaagatatgccaagaaa

SEQ ID NO: 4051 - RNA, 20 nt, synthetic construct
  source 1..20: mol_type = other RNA
atgccaagaaatggcatacc

SEQ ID NO: 4052 - RNA, 20 nt, synthetic construct
  source 1..20: mol_type = other RNA
atgcctggtatgccatttct

SEQ ID NO: 4053 - RNA, 20 nt, synthetic construct
  source 1..20: mol_type = other RNA
aatcatgtttataaaatgcc

SEQ ID NO: 4054 - RNA, 20 nt, synthetic construct
  source 1..20: mol_type = other RNA
attttataaacatgatttca

SEQ ID NO: 4055 - RNA, 20 nt, synthetic construct
  source 1..20: mol_type = other RNA
attcttctcaacaattttgc

SEQ ID NO: 4056 - RNA, 20 nt, synthetic construct
  source 1..20: mol_type = other RNA
aacaattttgctggaaattg

SEQ ID NO: 4057 - RNA, 20 nt, synthetic construct
  source 1..20: mol_type = other RNA
tgctggaaattgaggctcag

SEQ ID NO: 4058 - RNA, 20 nt, synthetic construct
  source 1..20: mol_type = other RNA
tcagaggaagcacttgccca

SEQ ID NO: 4059 - RNA, 20 nt, synthetic construct
  source 1..20: mol_type = other RNA
cagaggaagcacttgcccaa

SEQ ID NO: 4060 - RNA, 20 nt, synthetic construct
  source 1..20: mol_type = other RNA
caagggacataactagtaaa

SEQ ID NO: 4061 - RNA, 20 nt, synthetic construct
  source 1..20: mol_type = other RNA
atttactagttatgtccctt

SEQ ID NO: 4062 - RNA, 20 nt, synthetic construct
  source 1..20: mol_type = other RNA
ggacataactagtaaatggc

SEQ ID NO: 4063 - RNA, 20 nt, synthetic construct
  source 1..20: mol_type = other RNA
ggcaggtacagcacttacca

SEQ ID NO: 4064 - RNA, 20 nt, synthetic construct
  source 1..20: mol_type = other RNA
gcaggtacagcacttaccac

SEQ ID NO: 4065 - RNA, 20 nt, synthetic construct
  source 1..20: mol_type = other RNA
cttagagtgcagaagacccg

SEQ ID NO: 4066 - RNA, 20 nt, synthetic construct
  source 1..20: mol_type = other RNA
gtaaaaaaatacacgtagca

SEQ ID NO: 4067 - RNA, 20 nt, synthetic construct
  source 1..20: mol_type = other RNA
tacgtgtatttttttactga

SEQ ID NO: 4068 - RNA, 20 nt, synthetic construct
  source 1..20: mol_type = other RNA
aactgtctcaaaaactagtt

SEQ ID NO: 4069 - RNA, 20 nt, synthetic construct
  source 1..20: mol_type = other RNA
ttgagacagttaaaaataaa

SEQ ID NO: 4070 - RNA, 20 nt, synthetic construct
  source 1..20: mol_type = other RNA
aaaaaatatataaacattgt

SEQ ID NO: 4071 - RNA, 20 nt, synthetic construct
  source 1..20: mol_type = other RNA
tataaacattgttggttaag

SEQ ID NO: 4072 - RNA, 20 nt, synthetic construct
  source 1..20: mol_type = other RNA
cattcaaaattgctaattaa

SEQ ID NO: 4073 - RNA, 20 nt, synthetic construct
  source 1..20: mol_type = other RNA
gaatgatgaaacagccacat

SEQ ID NO: 4074 - RNA, 20 nt, synthetic construct
  source 1..20: mol_type = other RNA
ccacataggtgcaatgcttc

SEQ ID NO: 4075 - RNA, 20 nt, synthetic construct
  source 1..20: mol_type = other RNA
ccagaagcattgcacctatg

SEQ ID NO: 4076 - RNA, 20 nt, synthetic construct
  source 1..20: mol_type = other RNA
aggtgcaatgcttctggcca

SEQ ID NO: 4077 - RNA, 20 nt, synthetic construct
  source 1..20: mol_type = other RNA
tctggccagggcagctcatt

SEQ ID NO: 4078 - RNA, 20 nt, synthetic construct
  source 1..20: mol_type = other RNA
ctggccagggcagctcatta

SEQ ID NO: 4079 - RNA, 20 nt, synthetic construct
  source 1..20: mol_type = other RNA
gagtccctaatgagctgccc

SEQ ID NO: 4080 - RNA, 20 nt, synthetic construct
  source 1..20: mol_type = other RNA
ccgaagtctttctttttttt

SEQ ID NO: 4081 - RNA, 20 nt, synthetic construct
  source 1..20: mol_type = other RNA
agtctttctttttttttgga

SEQ ID NO: 4082 - RNA, 20 nt, synthetic construct
  source 1..20: mol_type = other RNA
ccaaaaaaaaagaaagactt

SEQ ID NO: 4083 - RNA, 20 nt, synthetic construct
  source 1..20: mol_type = other RNA
ggctatacagtgtgtataca

SEQ ID NO: 4084 - RNA, 20 nt, synthetic construct
  source 1..20: mol_type = other RNA
gtggtatgtaattttggtag

SEQ ID NO: 4085 - RNA, 20 nt, synthetic construct
  source 1..20: mol_type = other RNA
tgctaagtggtatgtaattt

SEQ ID NO: 4086 - RNA, 20 nt, synthetic construct
  source 1..20: mol_type = other RNA
tctcttgcattcgtgctaag

SEQ ID NO: 4087 - RNA, 20 nt, synthetic construct
  source 1..20: mol_type = other RNA
tttgtttatagtacgaggaa

SEQ ID NO: 4088 - RNA, 20 nt, synthetic construct
  source 1..20: mol_type = other RNA
ttttgtttatagtacgagga

SEQ ID NO: 4089 - RNA, 20 nt, synthetic construct
  source 1..20: mol_type = other RNA
taatttttgtttatagtacg

SEQ ID NO: 4090 - RNA, 20 nt, synthetic construct
  source 1..20: mol_type = other RNA
tagttttgtctcttacattt

SEQ ID NO: 4091 - RNA, 20 nt, synthetic construct
  source 1..20: mol_type = other RNA
ataaaactcttagaaaatat

SEQ ID NO: 4092 - RNA, 20 nt, synthetic construct
  source 1..20: mol_type = other RNA
taagaaggttttgctaatca

SEQ ID NO: 4093 - RNA, 20 nt, synthetic construct
  source 1..20: mol_type = other RNA
ttttcgtgtcatatctaaga

SEQ ID NO: 4094 - RNA, 20 nt, synthetic construct
  source 1..20: mol_type = other RNA
tcttttcaatttcttgataa

SEQ ID NO: 4095 - RNA, 20 nt, synthetic construct
  source 1..20: mol_type = other RNA
ttgaaaagatacacacagaa

SEQ ID NO: 4096 - RNA, 20 nt, synthetic construct
  source 1..20: mol_type = other RNA
tgaaaagatacacacagaat

SEQ ID NO: 4097 - RNA, 20 nt, synthetic construct
  source 1..20: mol_type = other RNA
tgtaaatcatgtatctgata

SEQ ID NO: 4098 - RNA, 20 nt, synthetic construct
  source 1..20: mol_type = other RNA
gtaaatcatgtatctgataa

SEQ ID NO: 4099 - RNA, 20 nt, synthetic construct
  source 1..20: mol_type = other RNA
aagaattcagtgtatatttc

SEQ ID NO: 4100 - RNA, 20 nt, synthetic construct
  source 1..20: mol_type = other RNA
atgtttgctcattttaaaat

SEQ ID NO: 4101 - RNA, 20 nt, synthetic construct
  source 1..20: mol_type = other RNA
ttaaaatgagcaaacattct

SEQ ID NO: 4102 - RNA, 20 nt, synthetic construct
  source 1..20: mol_type = other RNA
atgagcaaacattcttggcc

SEQ ID NO: 4103 - RNA, 20 nt, synthetic construct
  source 1..20: mol_type = other RNA
acattcttggccaggtgcaa

SEQ ID NO: 4104 - RNA, 20 nt, synthetic construct
  source 1..20: mol_type = other RNA
catgcatgagccattgcacc

SEQ ID NO: 4105 - RNA, 20 nt, synthetic construct
  source 1..20: mol_type = other RNA
tgcatgtaatcccagcactt

SEQ ID NO: 4106 - RNA, 20 nt, synthetic construct
  source 1..20: mol_type = other RNA
gcatgtaatcccagcacttt

SEQ ID NO: 4107 - RNA, 20 nt, synthetic construct
  source 1..20: mol_type = other RNA
tgtaatcccagcactttggg

SEQ ID NO: 4108 - RNA, 20 nt, synthetic construct
  source 1..20: mol_type = other RNA
cccagcactttgggaggcca

SEQ ID NO: 4109 - RNA, 20 nt, synthetic construct
  source 1..20: mol_type = other RNA
ccagcactttgggaggccaa

SEQ ID NO: 4110 - RNA, 20 nt, synthetic construct
  source 1..20: mol_type = other RNA
gcactttgggaggccaaggg

SEQ ID NO: 4111 - RNA, 20 nt, synthetic construct
  source 1..20: mol_type = other RNA
ccttggcctcccaaagtgct

SEQ ID NO: 4112 - RNA, 20 nt, synthetic construct
  source 1..20: mol_type = other RNA
cccttggcctcccaaagtgc

SEQ ID NO: 4113 - RNA, 20 nt, synthetic construct
  source 1..20: mol_type = other RNA
ctttgggaggccaagggagg

SEQ ID NO: 4114 - RNA, 20 nt, synthetic construct
  source 1..20: mol_type = other RNA
caagggaggtggatcacttg

SEQ ID NO: 4115 - RNA, 20 nt, synthetic construct
  source 1..20: mol_type = other RNA
ctcaagtgatccacctccct

SEQ ID NO: 4116 - RNA, 20 nt, synthetic construct
  source 1..20: mol_type = other RNA
gaggtggatcacttgaggtc

SEQ ID NO: 4117 - RNA, 20 nt, synthetic construct
  source 1..20: mol_type = other RNA
tcaggagttcaagaccagcc

SEQ ID NO: 4118 - RNA, 20 nt, synthetic construct
  source 1..20: mol_type = other RNA
caagaccagcctggccaaca

SEQ ID NO: 4119 - RNA, 20 nt, synthetic construct
  source 1..20: mol_type = other RNA
tttcaccatgttggccaggc

SEQ ID NO: 4120 - RNA, 20 nt, synthetic construct
  source 1..20: mol_type = other RNA
ggggtttcaccatgttggcc

SEQ ID NO: 4121 - RNA, 20 nt, synthetic construct
  source 1..20: mol_type = other RNA
gagatggggtttcaccatgt

SEQ ID NO: 4122 - RNA, 20 nt, synthetic construct
  source 1..20: mol_type = other RNA
ttgtatttttaatagagatg

SEQ ID NO: 4123 - RNA, 20 nt, synthetic construct
  source 1..20: mol_type = other RNA
tttgtatttttaatagagat

SEQ ID NO: 4124 - RNA, 20 nt, synthetic construct
  source 1..20: mol_type = other RNA
ttttgtatttttaatagaga

SEQ ID NO: 4125 - RNA, 20 nt, synthetic construct
  source 1..20: mol_type = other RNA
taaaaatacaaaaattagcc

SEQ ID NO: 4126 - RNA, 20 nt, synthetic construct
  source 1..20: mol_type = other RNA
atacaaaaattagccaggct

SEQ ID NO: 4127 - RNA, 20 nt, synthetic construct
  source 1..20: mol_type = other RNA
caaaaattagccaggcttgg

SEQ ID NO: 4128 - RNA, 20 nt, synthetic construct
  source 1..20: mol_type = other RNA
aaattagccaggcttggtgg

SEQ ID NO: 4129 - RNA, 20 nt, synthetic construct
  source 1..20: mol_type = other RNA
aattagccaggcttggtggt

SEQ ID NO: 4130 - RNA, 20 nt, synthetic construct
  source 1..20: mol_type = other RNA
caggcacccaccaccaagcc

SEQ ID NO: 4131 - RNA, 20 nt, synthetic construct
  source 1..20: mol_type = other RNA
tgcctgtaatctcagctact

SEQ ID NO: 4132 - RNA, 20 nt, synthetic construct
  source 1..20: mol_type = other RNA
gcctgtaatctcagctactt

SEQ ID NO: 4133 - RNA, 20 nt, synthetic construct
  source 1..20: mol_type = other RNA
tgtaatctcagctacttggg

SEQ ID NO: 4134 - RNA, 20 nt, synthetic construct
  source 1..20: mol_type = other RNA
tcccaagtagctgagattac

SEQ ID NO: 4135 - RNA, 20 nt, synthetic construct
  source 1..20: mol_type = other RNA
ctcagctacttgggaggctg

SEQ ID NO: 4136 - RNA, 20 nt, synthetic construct
  source 1..20: mol_type = other RNA
gctacttgggaggctgaggc

SEQ ID NO: 4137 - RNA, 20 nt, synthetic construct
  source 1..20: mol_type = other RNA
gcaggagaatagcttgaacc

SEQ ID NO: 4138 - RNA, 20 nt, synthetic construct
  source 1..20: mol_type = other RNA
caggagaatagcttgaacct

SEQ ID NO: 4139 - RNA, 20 nt, synthetic construct
  source 1..20: mol_type = other RNA
gagaatagcttgaacctggg

SEQ ID NO: 4140 - RNA, 20 nt, synthetic construct
  source 1..20: mol_type = other RNA
cactgtaggctctgcctccc

SEQ ID NO: 4141 - RNA, 20 nt, synthetic construct
  source 1..20: mol_type = other RNA
gcacgatcttggttcactgt

SEQ ID NO: 4142 - RNA, 20 nt, synthetic construct
  source 1..20: mol_type = other RNA
ggagtgcagtggcacgatct

SEQ ID NO: 4143 - RNA, 20 nt, synthetic construct
  source 1..20: mol_type = other RNA
cgtgccactgcactccagcc

SEQ ID NO: 4144 - RNA, 20 nt, synthetic construct
  source 1..20: mol_type = other RNA
gtgccactgcactccagcct

SEQ ID NO: 4145 - RNA, 20 nt, synthetic construct
  source 1..20: mol_type = other RNA
ttgcccaggctggagtgcag

SEQ ID NO: 4146 - RNA, 20 nt, synthetic construct
  source 1..20: mol_type = other RNA
ctcacttctgttgcccaggc

SEQ ID NO: 4147 - RNA, 20 nt, synthetic construct
  source 1..20: mol_type = other RNA
gagtctcacttctgttgccc

SEQ ID NO: 4148 - RNA, 20 nt, synthetic construct
  source 1..20: mol_type = other RNA
tttttttttttttttttttt

SEQ ID NO: 4149 - RNA, 20 nt, synthetic construct
  source 1..20: mol_type = other RNA
aaaaaaaaaaaaaaaagcaa

SEQ ID NO: 4150 - RNA, 20 nt, synthetic construct
  source 1..20: mol_type = other RNA
ctctaaagaagataaatgaa

SEQ ID NO: 4151 - RNA, 20 nt, synthetic construct
  source 1..20: mol_type = other RNA
aatgaatggcaaataagcac

SEQ ID NO: 4152 - RNA, 20 nt, synthetic construct
  source 1..20: mol_type = other RNA
tggcaaataagcacaggaaa

SEQ ID NO: 4153 - RNA, 20 nt, synthetic construct
  source 1..20: mol_type = other RNA
ttcaacatctttagtcttta

SEQ ID NO: 4154 - RNA, 20 nt, synthetic construct
  source 1..20: mol_type = other RNA
tgtgtggtggtgtctcattg

SEQ ID NO: 4155 - RNA, 20 nt, synthetic construct
  source 1..20: mol_type = other RNA
caccaccacacatgtagcat

SEQ ID NO: 4156 - RNA, 20 nt, synthetic construct
  source 1..20: mol_type = other RNA
accaccacacatgtagcatt

SEQ ID NO: 4157 - RNA, 20 nt, synthetic construct
  source 1..20: mol_type = other RNA
tcccaatgctacatgtgtgg

SEQ ID NO: 4158 - RNA, 20 nt, synthetic construct
  source 1..20: mol_type = other RNA
gcatcccaatgctacatgtg

SEQ ID NO: 4159 - RNA, 20 nt, synthetic construct
  source 1..20: mol_type = other RNA
attatgtgtctttttgatat

SEQ ID NO: 4160 - RNA, 20 nt, synthetic construct
  source 1..20: mol_type = other RNA
ataattaaaaagtcttagtg

SEQ ID NO: 4161 - RNA, 20 nt, synthetic construct
  source 1..20: mol_type = other RNA
aaaaagtcttagtgaggctg

SEQ ID NO: 4162 - RNA, 20 nt, synthetic construct
  source 1..20: mol_type = other RNA
tagtgaggctgtggagaaac

SEQ ID NO: 4163 - RNA, 20 nt, synthetic construct
  source 1..20: mol_type = other RNA
gaaccttcatacaccactag

SEQ ID NO: 4164 - RNA, 20 nt, synthetic construct
  source 1..20: mol_type = other RNA
aaccttcatacaccactagt

SEQ ID NO: 4165 - RNA, 20 nt, synthetic construct
  source 1..20: mol_type = other RNA
ctcccactagtggtgtatga

SEQ ID NO: 4166 - RNA, 20 nt, synthetic construct
  source 1..20: mol_type = other RNA
caccactagtgggagtttac

SEQ ID NO: 4167 - RNA, 20 nt, synthetic construct
  source 1..20: mol_type = other RNA
actagtgggagtttactggt

SEQ ID NO: 4168 - RNA, 20 nt, synthetic construct
  source 1..20: mol_type = other RNA
ctagtgggagtttactggta

SEQ ID NO: 4169 - RNA, 20 nt, synthetic construct
  source 1..20: mol_type = other RNA
taccagtaaactcccactag

SEQ ID NO: 4170 - RNA, 20 nt, synthetic construct
  source 1..20: mol_type = other RNA
gtaaagatattctaaaatta

SEQ ID NO: 4171 - RNA, 20 nt, synthetic construct
  source 1..20: mol_type = other RNA
atattctaaaattatggtga

SEQ ID NO: 4172 - RNA, 20 nt, synthetic construct
  source 1..20: mol_type = other RNA
atataaagtgtacaattcaa

SEQ ID NO: 4173 - RNA, 20 nt, synthetic construct
  source 1..20: mol_type = other RNA
ttgtacactttatatagatg

SEQ ID NO: 4174 - RNA, 20 nt, synthetic construct
  source 1..20: mol_type = other RNA
ctttatatagatgaggtgta

SEQ ID NO: 4175 - RNA, 20 nt, synthetic construct
  source 1..20: mol_type = other RNA
atatctgaatatagccagcg

SEQ ID NO: 4176 - RNA, 20 nt, synthetic construct
  source 1..20: mol_type = other RNA
ctttaaaacaacaaccacgc

SEQ ID NO: 4177 - RNA, 20 nt, synthetic construct
  source 1..20: mol_type = other RNA
ggttgttgttttaaagaaaa

SEQ ID NO: 4178 - RNA, 20 nt, synthetic construct
  source 1..20: mol_type = other RNA
cctcatttcttccaaatcca

SEQ ID NO: 4179 - RNA, 20 nt, synthetic construct
  source 1..20: mol_type = other RNA
ccttggatttggaagaaatg

SEQ ID NO: 4180 - RNA, 20 nt, synthetic construct
  source 1..20: mol_type = other RNA
aatccaaggcaagttagcaa

SEQ ID NO: 4181 - RNA, 20 nt, synthetic construct
  source 1..20: mol_type = other RNA
ttgctaacttgccttggatt

SEQ ID NO: 4182 - RNA, 20 nt, synthetic construct
  source 1..20: mol_type = other RNA
atgcctttgctaacttgcct

SEQ ID NO: 4183 - RNA, 20 nt, synthetic construct
  source 1..20: mol_type = other RNA
aaaggcataatgagaaaaag

SEQ ID NO: 4184 - RNA, 20 nt, synthetic construct
  source 1..20: mol_type = other RNA
gaggtctaattttcattcag

SEQ ID NO: 4185 - RNA, 20 nt, synthetic construct
  source 1..20: mol_type = other RNA
ggccacatcagtgctccatc

SEQ ID NO: 4186 - RNA, 20 nt, synthetic construct
  source 1..20: mol_type = other RNA
gtccagatggagcactgatg

SEQ ID NO: 4187 - RNA, 20 nt, synthetic construct
  source 1..20: mol_type = other RNA
tggctgactctttgtccaga

SEQ ID NO: 4188 - RNA, 20 nt, synthetic construct
  source 1..20: mol_type = other RNA
cagccaagaagccaactgcc

SEQ ID NO: 4189 - RNA, 20 nt, synthetic construct
  source 1..20: mol_type = other RNA
aagaagccaactgccaggag

SEQ ID NO: 4190 - RNA, 20 nt, synthetic construct
  source 1..20: mol_type = other RNA
actcctggcagttggcttct

SEQ ID NO: 4191 - RNA, 20 nt, synthetic construct
  source 1..20: mol_type = other RNA
catcttccactcctggcagt

SEQ ID NO: 4192 - RNA, 20 nt, synthetic construct
  source 1..20: mol_type = other RNA
aagtggtcatcttccactcc

SEQ ID NO: 4193 - RNA, 20 nt, synthetic construct
  source 1..20: mol_type = other RNA
agatgaccacttccaggatc

SEQ ID NO: 4194 - RNA, 20 nt, synthetic construct
  source 1..20: mol_type = other RNA
tctctgccagatcctggaag

SEQ ID NO: 4195 - RNA, 20 nt, synthetic construct
  source 1..20: mol_type = other RNA
aaagtctctctgccagatcc

SEQ ID NO: 4196 - RNA, 20 nt, synthetic construct
  source 1..20: mol_type = other RNA
tttgcaagtgcctttgaaag

SEQ ID NO: 4197 - RNA, 20 nt, synthetic construct
  source 1..20: mol_type = other RNA
ttttcattgtcctctttcaa

SEQ ID NO: 4198 - RNA, 20 nt, synthetic construct
  source 1..20: mol_type = other RNA
gaggacaatgaaaatgtatc

SEQ ID NO: 4199 - RNA, 20 nt, synthetic construct
  source 1..20: mol_type = other RNA
tatctggcatgaaacacagc

SEQ ID NO: 4200 - RNA, 20 nt, synthetic construct
  source 1..20: mol_type = other RNA
cacagcaggatccaaagaac

SEQ ID NO: 4201 - RNA, 20 nt, synthetic construct
  source 1..20: mol_type = other RNA
caatatcaaagcctgttctt

SEQ ID NO: 4202 - RNA, 20 nt, synthetic construct
  source 1..20: mol_type = other RNA
ttaaagacacgcatcatgac

SEQ ID NO: 4203 - RNA, 20 nt, synthetic construct
  source 1..20: mol_type = other RNA
agaaggatacacttagtcat

SEQ ID NO: 4204 - RNA, 20 nt, synthetic construct
  source 1..20: mol_type = other RNA
ctgcacacgagtggatcaga

SEQ ID NO: 4205 - RNA, 20 nt, synthetic construct
  source 1..20: mol_type = other RNA
gttctctaactgcacacgag

SEQ ID NO: 4206 - RNA, 20 nt, synthetic construct
  source 1..20: mol_type = other RNA
gtgcagttagagaacaccca

SEQ ID NO: 4207 - RNA, 20 nt, synthetic construct
  source 1..20: mol_type = other RNA
tgcagttagagaacacccaa

SEQ ID NO: 4208 - RNA, 20 nt, synthetic construct
  source 1..20: mol_type = other RNA
gcagttagagaacacccaag

SEQ ID NO: 4209 - RNA, 20 nt, synthetic construct
  source 1..20: mol_type = other RNA
gtgtgtgtgtgggacccctt

SEQ ID NO: 4210 - RNA, 20 nt, synthetic construct
  source 1..20: mol_type = other RNA
cgtgtgtgtgtgggacccct

SEQ ID NO: 4211 - RNA, 20 nt, synthetic construct
  source 1..20: mol_type = other RNA
ggtcccacacacacacgtga

SEQ ID NO: 4212 - RNA, 20 nt, synthetic construct
  source 1..20: mol_type = other RNA
gtcccacacacacacgtgaa

SEQ ID NO: 4213 - RNA, 20 nt, synthetic construct
  source 1..20: mol_type = other RNA
tcccacacacacacgtgaag

SEQ ID NO: 4214 - RNA, 20 nt, synthetic construct
  source 1..20: mol_type = other RNA
tccccttcacgtgtgtgtgt

SEQ ID NO: 4215 - RNA, 20 nt, synthetic construct
  source 1..20: mol_type = other RNA
gtccccttcacgtgtgtgtg

SEQ ID NO: 4216 - RNA, 20 nt, synthetic construct
  source 1..20: mol_type = other RNA
ggggacactcccaacccatg

SEQ ID NO: 4217 - RNA, 20 nt, synthetic construct
  source 1..20: mol_type = other RNA
gggacactcccaacccatga

SEQ ID NO: 4218 - RNA, 20 nt, synthetic construct
  source 1..20: mol_type = other RNA
gtgtgtttccctcatgggtt

SEQ ID NO: 4219 - RNA, 20 nt, synthetic construct
  source 1..20: mol_type = other RNA
ggtgtgtttccctcatgggt

SEQ ID NO: 4220 - RNA, 20 nt, synthetic construct
  source 1..20: mol_type = other RNA
ggagggtgtgtttccctcat

SEQ ID NO: 4221 - RNA, 20 nt, synthetic construct
  source 1..20: mol_type = other RNA
tggagggtgtgtttccctca

SEQ ID NO: 4222 - RNA, 20 nt, synthetic construct
  source 1..20: mol_type = other RNA
acacaccctccatcctcctt

SEQ ID NO: 4223 - RNA, 20 nt, synthetic construct
  source 1..20: mol_type = other RNA
ttgaaccaaaggaggatgga

SEQ ID NO: 4224 - RNA, 20 nt, synthetic construct
  source 1..20: mol_type = other RNA
gttgaaccaaaggaggatgg

SEQ ID NO: 4225 - RNA, 20 nt, synthetic construct
  source 1..20: mol_type = other RNA
ggggttgaaccaaaggagga

SEQ ID NO: 4226 - RNA, 20 nt, synthetic construct
  source 1..20: mol_type = other RNA
ggctggggttgaaccaaagg

SEQ ID NO: 4227 - RNA, 20 nt, synthetic construct
  source 1..20: mol_type = other RNA
ggaggctggggttgaaccaa

SEQ ID NO: 4228 - RNA, 20 nt, synthetic construct
  source 1..20: mol_type = other RNA
caaccccagcctccgagaac

SEQ ID NO: 4229 - RNA, 20 nt, synthetic construct
  source 1..20: mol_type = other RNA
ttacctgttctcggaggctg

SEQ ID NO: 4230 - RNA, 20 nt, synthetic construct
  source 1..20: mol_type = other RNA
attacctgttctcggaggct

SEQ ID NO: 4231 - RNA, 20 nt, synthetic construct
  source 1..20: mol_type = other RNA
aattacctgttctcggaggc

SEQ ID NO: 4232 - RNA, 20 nt, synthetic construct
  source 1..20: mol_type = other RNA
ccgagaacaggtaatttcat

SEQ ID NO: 4233 - RNA, 20 nt, synthetic construct
  source 1..20: mol_type = other RNA
atgaaattacctgttctcgg

SEQ ID NO: 4234 - RNA, 20 nt, synthetic construct
  source 1..20: mol_type = other RNA
cctatgaaattacctgttct

SEQ ID NO: 4235 - RNA, 20 nt, synthetic construct
  source 1..20: mol_type = other RNA
ctataaaggtgacaagtttg

SEQ ID NO: 4236 - RNA, 20 nt, synthetic construct
  source 1..20: mol_type = other RNA
ttatagtcacttgaagaagt

SEQ ID NO: 4237 - RNA, 20 nt, synthetic construct
  source 1..20: mol_type = other RNA
acttcttcaagtgactataa

SEQ ID NO: 4238 - RNA, 20 nt, synthetic construct
  source 1..20: mol_type = other RNA
gaaaaatacagtgaaagtcc

SEQ ID NO: 4239 - RNA, 20 nt, synthetic construct
  source 1..20: mol_type = other RNA
tacatctctgttgtagcacc

SEQ ID NO: 4240 - RNA, 20 nt, synthetic construct
  source 1..20: mol_type = other RNA
atgtaaagcttatctggcat

SEQ ID NO: 4241 - RNA, 20 nt, synthetic construct
  source 1..20: mol_type = other RNA
taacacatgtaaagcttatc

SEQ ID NO: 4242 - RNA, 20 nt, synthetic construct
  source 1..20: mol_type = other RNA
cctcattagtcactcaacac

SEQ ID NO: 4243 - RNA, 20 nt, synthetic construct
  source 1..20: mol_type = other RNA
ctcattagtcactcaacaca

SEQ ID NO: 4244 - RNA, 20 nt, synthetic construct
  source 1..20: mol_type = other RNA
cctgtgttgagtgactaatg

SEQ ID NO: 4245 - RNA, 20 nt, synthetic construct
  source 1..20: mol_type = other RNA
acacagggtgatcatcttac

SEQ ID NO: 4246 - RNA, 20 nt, synthetic construct
  source 1..20: mol_type = other RNA
tcttacaggaagagatactg

SEQ ID NO: 4247 - RNA, 20 nt, synthetic construct
  source 1..20: mol_type = other RNA
aggaagagatactgaggcac

SEQ ID NO: 4248 - RNA, 20 nt, synthetic construct
  source 1..20: mol_type = other RNA
caggaatgtcaacttgccta

SEQ ID NO: 4249 - RNA, 20 nt, synthetic construct
  source 1..20: mol_type = other RNA
cctaaggtcacaaagctaga

SEQ ID NO: 4250 - RNA, 20 nt, synthetic construct
  source 1..20: mol_type = other RNA
ccttctagctttgtgacctt

SEQ ID NO: 4251 - RNA, 20 nt, synthetic construct
  source 1..20: mol_type = other RNA
aaagctagaaggaacaaaat

SEQ ID NO: 4252 - RNA, 20 nt, synthetic construct
  source 1..20: mol_type = other RNA
aagctagaaggaacaaaata

SEQ ID NO: 4253 - RNA, 20 nt, synthetic construct
  source 1..20: mol_type = other RNA
ggcttcaaacccagtcattt

SEQ ID NO: 4254 - RNA, 20 nt, synthetic construct
  source 1..20: mol_type = other RNA
cccagtcattttggctccaa

SEQ ID NO: 4255 - RNA, 20 nt, synthetic construct
  source 1..20: mol_type = other RNA
cctttggagccaaaatgact

SEQ ID NO: 4256 - RNA, 20 nt, synthetic construct
  source 1..20: mol_type = other RNA
gcctttggagccaaaatgac

SEQ ID NO: 4257 - RNA, 20 nt, synthetic construct
  source 1..20: mol_type = other RNA
agtggttaaggcatagcctt

SEQ ID NO: 4258 - RNA, 20 nt, synthetic construct
  source 1..20: mol_type = other RNA
ggcgcttagcacagtggtta

SEQ ID NO: 4259 - RNA, 20 nt, synthetic construct
  source 1..20: mol_type = other RNA
gcaggcggcgcttagcacag

SEQ ID NO: 4260 - RNA, 20 nt, synthetic construct
  source 1..20: mol_type = other RNA
ctaagcgccgcctgcttaac

SEQ ID NO: 4261 - RNA, 20 nt, synthetic construct
  source 1..20: mol_type = other RNA
taagcgccgcctgcttaacc

SEQ ID NO: 4262 - RNA, 20 nt, synthetic construct
  source 1..20: mol_type = other RNA
aggtagcccggttaagcagg

SEQ ID NO: 4263 - RNA, 20 nt, synthetic construct
  source 1..20: mol_type = other RNA
aaaaggtagcccggttaagc

SEQ ID NO: 4264 - RNA, 20 nt, synthetic construct
  source 1..20: mol_type = other RNA
ttgtggtggaaaaggtagcc

SEQ ID NO: 4265 - RNA, 20 nt, synthetic construct
  source 1..20: mol_type = other RNA
atgagaaattgtggtggaaa

SEQ ID NO: 4266 - RNA, 20 nt, synthetic construct
  source 1..20: mol_type = other RNA
gaagggatgagaaattgtgg

SEQ ID NO: 4267 - RNA, 20 nt, synthetic construct
  source 1..20: mol_type = other RNA
tcagaagggatgagaaattg

SEQ ID NO: 4268 - RNA, 20 nt, synthetic construct
  source 1..20: mol_type = other RNA
ttctcatcccttctgaaaga

SEQ ID NO: 4269 - RNA, 20 nt, synthetic construct
  source 1..20: mol_type = other RNA
cccttctgaaagatggtcac

SEQ ID NO: 4270 - RNA, 20 nt, synthetic construct
  source 1..20: mol_type = other RNA
cctgtgaccatctttcagaa

SEQ ID NO: 4271 - RNA, 20 nt, synthetic construct
  source 1..20: mol_type = other RNA
acctgtgaccatctttcaga

SEQ ID NO: 4272 - RNA, 20 nt, synthetic construct
  source 1..20: mol_type = other RNA
cacaggtgttgctgaaatac

SEQ ID NO: 4273 - RNA, 20 nt, synthetic construct
  source 1..20: mol_type = other RNA
ttttaaatagttttacattt

SEQ ID NO: 4274 - RNA, 20 nt, synthetic construct
  source 1..20: mol_type = other RNA
tttaaatagttttacattta

SEQ ID NO: 4275 - RNA, 20 nt, synthetic construct
  source 1..20: mol_type = other RNA
ttaaatagttttacatttag

SEQ ID NO: 4276 - RNA, 20 nt, synthetic construct
  source 1..20: mol_type = other RNA
cttgtatacccctcaccccc

SEQ ID NO: 4277 - RNA, 20 nt, synthetic construct
  source 1..20: mol_type = other RNA
agggggtgaggggtatacaa

SEQ ID NO: 4278 - RNA, 20 nt, synthetic construct
  source 1..20: mol_type = other RNA
cagggggtgaggggtataca

SEQ ID NO: 4279 - RNA, 20 nt, synthetic construct
  source 1..20: mol_type = other RNA
aggggtatccagggggtgag

SEQ ID NO: 4280 - RNA, 20 nt, synthetic construct
  source 1..20: mol_type = other RNA
gaggggtatccagggggtga

SEQ ID NO: 4281 - RNA, 20 nt, synthetic construct
  source 1..20: mol_type = other RNA
tgaggggtatccagggggtg

SEQ ID NO: 4282 - RNA, 20 nt, synthetic construct
  source 1..20: mol_type = other RNA
ccaagtgaggggtatccagg

SEQ ID NO: 4283 - RNA, 20 nt, synthetic construct
  source 1..20: mol_type = other RNA
accaagtgaggggtatccag

SEQ ID NO: 4284 - RNA, 20 nt, synthetic construct
  source 1..20: mol_type = other RNA
aaccaagtgaggggtatcca

SEQ ID NO: 4285 - RNA, 20 nt, synthetic construct
  source 1..20: mol_type = other RNA
aaaccaagtgaggggtatcc

SEQ ID NO: 4286 - RNA, 20 nt, synthetic construct
  source 1..20: mol_type = other RNA
aacagaataaaccaagtgag

SEQ ID NO: 4287 - RNA, 20 nt, synthetic construct
  source 1..20: mol_type = other RNA
caacagaataaaccaagtga

SEQ ID NO: 4288 - RNA, 20 nt, synthetic construct
  source 1..20: mol_type = other RNA
acaacagaataaaccaagtg

SEQ ID NO: 4289 - RNA, 20 nt, synthetic construct
  source 1..20: mol_type = other RNA
gatgtacgtagtaatgtcaa

SEQ ID NO: 4290 - RNA, 20 nt, synthetic construct
  source 1..20: mol_type = other RNA
tacgtacatctgtcacaatg

SEQ ID NO: 4291 - RNA, 20 nt, synthetic construct
  source 1..20: mol_type = other RNA
acgtacatctgtcacaatga

SEQ ID NO: 4292 - RNA, 20 nt, synthetic construct
  source 1..20: mol_type = other RNA
tacatctgtcacaatgaggg

SEQ ID NO: 4293 - RNA, 20 nt, synthetic construct
  source 1..20: mol_type = other RNA
cacaatgagggaggcaacac

SEQ ID NO: 4294 - RNA, 20 nt, synthetic construct
  source 1..20: mol_type = other RNA
actacacgctacactttctt

SEQ ID NO: 4295 - RNA, 20 nt, synthetic construct
  source 1..20: mol_type = other RNA
ggacagaaaaggacattaag

SEQ ID NO: 4296 - RNA, 20 nt, synthetic construct
  source 1..20: mol_type = other RNA
gggacagaaaaggacattaa

SEQ ID NO: 4297 - RNA, 20 nt, synthetic construct
  source 1..20: mol_type = other RNA
tgggacagaaaaggacatta

SEQ ID NO: 4298 - RNA, 20 nt, synthetic construct
  source 1..20: mol_type = other RNA
atgggatcttgggacagaaa

SEQ ID NO: 4299 - RNA, 20 nt, synthetic construct
  source 1..20: mol_type = other RNA
acgtagtgggatgggatctt

SEQ ID NO: 4300 - RNA, 20 nt, synthetic construct
  source 1..20: mol_type = other RNA
aacgtagtgggatgggatct

SEQ ID NO: 4301 - RNA, 20 nt, synthetic construct
  source 1..20: mol_type = other RNA
agctctaaacgtagtgggat

SEQ ID NO: 4302 - RNA, 20 nt, synthetic construct
  source 1..20: mol_type = other RNA
gagctctaaacgtagtggga

SEQ ID NO: 4303 - RNA, 20 nt, synthetic construct
  source 1..20: mol_type = other RNA
ccatgagctctaaacgtagt

SEQ ID NO: 4304 - RNA, 20 nt, synthetic construct
  source 1..20: mol_type = other RNA
gccatgagctctaaacgtag

SEQ ID NO: 4305 - RNA, 20 nt, synthetic construct
  source 1..20: mol_type = other RNA
gagctcatggctcctttgcc

SEQ ID NO: 4306 - RNA, 20 nt, synthetic construct
  source 1..20: mol_type = other RNA
catggctcctttgcctggcc

SEQ ID NO: 4307 - RNA, 20 nt, synthetic construct
  source 1..20: mol_type = other RNA
tcactgaccaggccaggcaa

SEQ ID NO: 4308 - RNA, 20 nt, synthetic construct
  source 1..20: mol_type = other RNA
aaagtgtcactgaccaggcc

SEQ ID NO: 4309 - RNA, 20 nt, synthetic construct
  source 1..20: mol_type = other RNA
tgagcaaagtgtcactgacc

SEQ ID NO: 4310 - RNA, 20 nt, synthetic construct
  source 1..20: mol_type = other RNA
cttgttttcgatgacgttga

SEQ ID NO: 4311 - RNA, 20 nt, synthetic construct
  source 1..20: mol_type = other RNA
atcaacgtcatcgaaaacaa

SEQ ID NO: 4312 - RNA, 20 nt, synthetic construct
  source 1..20: mol_type = other RNA
catcaacgtcatcgaaaaca

SEQ ID NO: 4313 - RNA, 20 nt, synthetic construct
  source 1..20: mol_type = other RNA
cgatgacgttgatggtcttg

SEQ ID NO: 4314 - RNA, 20 nt, synthetic construct
  source 1..20: mol_type = other RNA
tggtcttgaggaacactgcc

SEQ ID NO: 4315 - RNA, 20 nt, synthetic construct
  source 1..20: mol_type = other RNA
gaggaacactgccaggcatt

SEQ ID NO: 4316 - RNA, 20 nt, synthetic construct
  source 1..20: mol_type = other RNA
gggatattttaccaaatgcc

SEQ ID NO: 4317 - RNA, 20 nt, synthetic construct
  source 1..20: mol_type = other RNA
ggtaaaatatccctcaatgt

SEQ ID NO: 4318 - RNA, 20 nt, synthetic construct
  source 1..20: mol_type = other RNA
atcagtcaaacctacattga

SEQ ID NO: 4319 - RNA, 20 nt, synthetic construct
  source 1..20: mol_type = other RNA
catcagtcaaacctacattg

SEQ ID NO: 4320 - RNA, 20 nt, synthetic construct
  source 1..20: mol_type = other RNA
tcatcactagacccagatta

SEQ ID NO: 4321 - RNA, 20 nt, synthetic construct
  source 1..20: mol_type = other RNA
catcactagacccagattat

SEQ ID NO: 4322 - RNA, 20 nt, synthetic construct
  source 1..20: mol_type = other RNA
acccagattatgggtttttc

SEQ ID NO: 4323 - RNA, 20 nt, synthetic construct
  source 1..20: mol_type = other RNA
acctgaaaaacccataatct

SEQ ID NO: 4324 - RNA, 20 nt, synthetic construct
  source 1..20: mol_type = other RNA
gacctgaaaaacccataatc

SEQ ID NO: 4325 - RNA, 20 nt, synthetic construct
  source 1..20: mol_type = other RNA
cttctcaccacatcctgtca

SEQ ID NO: 4326 - RNA, 20 nt, synthetic construct
  source 1..20: mol_type = other RNA
cttgacaggatgtggtgaga

SEQ ID NO: 4327 - RNA, 20 nt, synthetic construct
  source 1..20: mol_type = other RNA
tgtcacaccttgacaggatg

SEQ ID NO: 4328 - RNA, 20 nt, synthetic construct
  source 1..20: mol_type = other RNA
cgactatgtcacaccttgac

SEQ ID NO: 4329 - RNA, 20 nt, synthetic construct
  source 1..20: mol_type = other RNA
agtcgatgtgaactgatcac

SEQ ID NO: 4330 - RNA, 20 nt, synthetic construct
  source 1..20: mol_type = other RNA
gtcgatgtgaactgatcact

SEQ ID NO: 4331 - RNA, 20 nt, synthetic construct
  source 1..20: mol_type = other RNA
gggatgagaaactgtttgcc

SEQ ID NO: 4332 - RNA, 20 nt, synthetic construct
  source 1..20: mol_type = other RNA
aacttagaggtggagaaacc

SEQ ID NO: 4333 - RNA, 20 nt, synthetic construct
  source 1..20: mol_type = other RNA
gaaagaaagtaacttagagg

SEQ ID NO: 4334 - RNA, 20 nt, synthetic construct
  source 1..20: mol_type = other RNA
aaggaaagaaagtaacttag

SEQ ID NO: 4335 - RNA, 20 nt, synthetic construct
  source 1..20: mol_type = other RNA
tcaaacatcacactagggca

SEQ ID NO: 4336 - RNA, 20 nt, synthetic construct
  source 1..20: mol_type = other RNA
tagcttcaaacatcacacta

SEQ ID NO: 4337 - RNA, 20 nt, synthetic construct
  source 1..20: mol_type = other RNA
ttagcttcaaacatcacact

SEQ ID NO: 4338 - RNA, 20 nt, synthetic construct
  source 1..20: mol_type = other RNA
caaagtgcagcccatgctgt

SEQ ID NO: 4339 - RNA, 20 nt, synthetic construct
  source 1..20: mol_type = other RNA
tacagcatgggctgcacttt

SEQ ID NO: 4340 - RNA, 20 nt, synthetic construct
  source 1..20: mol_type = other RNA
ctacagcatgggctgcactt

SEQ ID NO: 4341 - RNA, 20 nt, synthetic construct
  source 1..20: mol_type = other RNA
cagcccatgctgtaggaatg

SEQ ID NO: 4342 - RNA, 20 nt, synthetic construct
  source 1..20: mol_type = other RNA
actcctcattcctacagcat

SEQ ID NO: 4343 - RNA, 20 nt, synthetic construct
  source 1..20: mol_type = other RNA
aactcctcattcctacagca

SEQ ID NO: 4344 - RNA, 20 nt, synthetic construct
  source 1..20: mol_type = other RNA
gttaagctccatctccttaa

SEQ ID NO: 4345 - RNA, 20 nt, synthetic construct
  source 1..20: mol_type = other RNA
ttaagctccatctccttaat

SEQ ID NO: 4346 - RNA, 20 nt, synthetic construct
  source 1..20: mol_type = other RNA
taagctccatctccttaatg

SEQ ID NO: 4347 - RNA, 20 nt, synthetic construct
  source 1..20: mol_type = other RNA
gttactccccattaaggaga

SEQ ID NO: 4348 - RNA, 20 nt, synthetic construct
  source 1..20: mol_type = other RNA
tatatagttactccccatta

SEQ ID NO: 4349 - RNA, 20 nt, synthetic construct
  source 1..20: mol_type = other RNA
tataaccttatttttaatga

SEQ ID NO: 4350 - RNA, 20 nt, synthetic construct
  source 1..20: mol_type = other RNA
attaaccatcattaaaaata

SEQ ID NO: 4351 - RNA, 20 nt, synthetic construct
  source 1..20: mol_type = other RNA
ttaatgatggttaatccgta

SEQ ID NO: 4352 - RNA, 20 nt, synthetic construct
  source 1..20: mol_type = other RNA
ttattttttttaatgccata

SEQ ID NO: 4353 - RNA, 20 nt, synthetic construct
  source 1..20: mol_type = other RNA
acatgccaagtgacagtgta

SEQ ID NO: 4354 - RNA, 20 nt, synthetic construct
  source 1..20: mol_type = other RNA
aagggccgtacactgtcact

SEQ ID NO: 4355 - RNA, 20 nt, synthetic construct
  source 1..20: mol_type = other RNA
gagtcagcaacaatagggaa

SEQ ID NO: 4356 - RNA, 20 nt, synthetic construct
  source 1..20: mol_type = other RNA
agagtcagcaacaataggga

SEQ ID NO: 4357 - RNA, 20 nt, synthetic construct
  source 1..20: mol_type = other RNA
tattgttgctgactctgcag

SEQ ID NO: 4358 - RNA, 20 nt, synthetic construct
  source 1..20: mol_type = other RNA
ctgcagagtcagcaacaata

SEQ ID NO: 4359 - RNA, 20 nt, synthetic construct
  source 1..20: mol_type = other RNA
actgcagagtcagcaacaat

SEQ ID NO: 4360 - RNA, 20 nt, synthetic construct
  source 1..20: mol_type = other RNA
tgactctgcagtggctgtaa

SEQ ID NO: 4361 - RNA, 20 nt, synthetic construct
  source 1..20: mol_type = other RNA
tctgagacataaagatgatc

SEQ ID NO: 4362 - RNA, 20 nt, synthetic construct
  source 1..20: mol_type = other RNA
tctttatgtctcagaatcac

SEQ ID NO: 4363 - RNA, 20 nt, synthetic construct
  source 1..20: mol_type = other RNA
ttatgtctcagaatcacagg

SEQ ID NO: 4364 - RNA, 20 nt, synthetic construct
  source 1..20: mol_type = other RNA
ggtaagaagcactatctcca

SEQ ID NO: 4365 - RNA, 20 nt, synthetic construct
  source 1..20: mol_type = other RNA
gttttacttttttgtcacct

SEQ ID NO: 4366 - RNA, 20 nt, synthetic construct
  source 1..20: mol_type = other RNA
tgacaaaaaagtaaaacaac

SEQ ID NO: 4367 - RNA, 20 nt, synthetic construct
  source 1..20: mol_type = other RNA
agtaaaacaactggccagca

SEQ ID NO: 4368 - RNA, 20 nt, synthetic construct
  source 1..20: mol_type = other RNA
caactggccagcatggaaag

SEQ ID NO: 4369 - RNA, 20 nt, synthetic construct
  source 1..20: mol_type = other RNA
aactggccagcatggaaaga

SEQ ID NO: 4370 - RNA, 20 nt, synthetic construct
  source 1..20: mol_type = other RNA
ggacttccctctttccatgc

SEQ ID NO: 4371 - RNA, 20 nt, synthetic construct
  source 1..20: mol_type = other RNA
aaacatcatctagaatggaa

SEQ ID NO: 4372 - RNA, 20 nt, synthetic construct
  source 1..20: mol_type = other RNA
ttgttaaacatcatctagaa

SEQ ID NO: 4373 - RNA, 20 nt, synthetic construct
  source 1..20: mol_type = other RNA
gatgatgtttaacaaacaac

SEQ ID NO: 4374 - RNA, 20 nt, synthetic construct
  source 1..20: mol_type = other RNA
aaacaacaggagtcagagaa

SEQ ID NO: 4375 - RNA, 20 nt, synthetic construct
  source 1..20: mol_type = other RNA
gagaaaaaactatcccatga

SEQ ID NO: 4376 - RNA, 20 nt, synthetic construct
  source 1..20: mol_type = other RNA
aaaaaactatcccatgatgg

SEQ ID NO: 4377 - RNA, 20 nt, synthetic construct
  source 1..20: mol_type = other RNA
gcatgtgttgcctccatcat

SEQ ID NO: 4378 - RNA, 20 nt, synthetic construct
  source 1..20: mol_type = other RNA
agcatgtgttgcctccatca

SEQ ID NO: 4379 - RNA, 20 nt, synthetic construct
  source 1..20: mol_type = other RNA
acacatgctgcatgtttgta

SEQ ID NO: 4380 - RNA, 20 nt, synthetic construct
  source 1..20: mol_type = other RNA
cacatgctgcatgtttgtat

SEQ ID NO: 4381 - RNA, 20 nt, synthetic construct
  source 1..20: mol_type = other RNA
tgctgcatgtttgtatgggc

SEQ ID NO: 4382 - RNA, 20 nt, synthetic construct
  source 1..20: mol_type = other RNA
tgtatgggcaggtattaaac

SEQ ID NO: 4383 - RNA, 20 nt, synthetic construct
  source 1..20: mol_type = other RNA
aatttatatctgtcattgct

SEQ ID NO: 4384 - RNA, 20 nt, synthetic construct
  source 1..20: mol_type = other RNA
agatataaatttccaaagtg

SEQ ID NO: 4385 - RNA, 20 nt, synthetic construct
  source 1..20: mol_type = other RNA
aatttccaaagtgaggtgcc

SEQ ID NO: 4386 - RNA, 20 nt, synthetic construct
  source 1..20: mol_type = other RNA
gagagcctggcacctcactt

SEQ ID NO: 4387 - RNA, 20 nt, synthetic construct
  source 1..20: mol_type = other RNA
tgaggtgccaggctctccaa

SEQ ID NO: 4388 - RNA, 20 nt, synthetic construct
  source 1..20: mol_type = other RNA
aaaagctcctttggagagcc

SEQ ID NO: 4389 - RNA, 20 nt, synthetic construct
  source 1..20: mol_type = other RNA
ttaactttgaaaagctcctt

SEQ ID NO: 4390 - RNA, 20 nt, synthetic construct
  source 1..20: mol_type = other RNA
ttctcactcagagtaggtcg

SEQ ID NO: 4391 - RNA, 20 nt, synthetic construct
  source 1..20: mol_type = other RNA
tttctcactcagagtaggtc

SEQ ID NO: 4392 - RNA, 20 nt, synthetic construct
  source 1..20: mol_type = other RNA
gtttctcactcagagtaggt

SEQ ID NO: 4393 - RNA, 20 nt, synthetic construct
  source 1..20: mol_type = other RNA
ttctgtttctcactcagagt

SEQ ID NO: 4394 - RNA, 20 nt, synthetic construct
  source 1..20: mol_type = other RNA
gagaattttgtttttctttg

SEQ ID NO: 4395 - RNA, 20 nt, synthetic construct
  source 1..20: mol_type = other RNA
agaattttgtttttctttga

SEQ ID NO: 4396 - RNA, 20 nt, synthetic construct
  source 1..20: mol_type = other RNA
gaattttgtttttctttgag

SEQ ID NO: 4397 - RNA, 20 nt, synthetic construct
  source 1..20: mol_type = other RNA
aattttgtttttctttgagg

SEQ ID NO: 4398 - RNA, 20 nt, synthetic construct
  source 1..20: mol_type = other RNA
ctccaccatcaccaaagaga

SEQ ID NO: 4399 - RNA, 20 nt, synthetic construct
  source 1..20: mol_type = other RNA
tccaccatcaccaaagagat

SEQ ID NO: 4400 - RNA, 20 nt, synthetic construct
  source 1..20: mol_type = other RNA
tctctttggtgatggtggag

SEQ ID NO: 4401 - RNA, 20 nt, synthetic construct
  source 1..20: mol_type = other RNA
atctctttggtgatggtgga

SEQ ID NO: 4402 - RNA, 20 nt, synthetic construct
  source 1..20: mol_type = other RNA
catctctttggtgatggtgg

SEQ ID NO: 4403 - RNA, 20 nt, synthetic construct
  source 1..20: mol_type = other RNA
acccatctctttggtgatgg

SEQ ID NO: 4404 - RNA, 20 nt, synthetic construct
  source 1..20: mol_type = other RNA
gctacccatctctttggtga

SEQ ID NO: 4405 - RNA, 20 nt, synthetic construct
  source 1..20: mol_type = other RNA
caaagagatgggtagcacag

SEQ ID NO: 4406 - RNA, 20 nt, synthetic construct
  source 1..20: mol_type = other RNA
agagatgggtagcacagtgg

SEQ ID NO: 4407 - RNA, 20 nt, synthetic construct
  source 1..20: mol_type = other RNA
gagatgggtagcacagtgga

SEQ ID NO: 4408 - RNA, 20 nt, synthetic construct
  source 1..20: mol_type = other RNA
agatgggtagcacagtggag

SEQ ID NO: 4409 - RNA, 20 nt, synthetic construct
  source 1..20: mol_type = other RNA
gatgggtagcacagtggagg

SEQ ID NO: 4410 - RNA, 20 nt, synthetic construct
  source 1..20: mol_type = other RNA
atgggtagcacagtggaggg

SEQ ID NO: 4411 - RNA, 20 nt, synthetic construct
  source 1..20: mol_type = other RNA
tgggtagcacagtggagggg

SEQ ID NO: 4412 - RNA, 20 nt, synthetic construct
  source 1..20: mol_type = other RNA
gggtagcacagtggaggggg

SEQ ID NO: 4413 - RNA, 20 nt, synthetic construct
  source 1..20: mol_type = other RNA
ggtagcacagtggagggggg

SEQ ID NO: 4414 - RNA, 20 nt, synthetic construct
  source 1..20: mol_type = other RNA
gtagcacagtggaggggggg

SEQ ID NO: 4415 - RNA, 20 nt, synthetic construct
  source 1..20: mol_type = other RNA
tagcacagtggagggggggg

SEQ ID NO: 4416 - RNA, 20 nt, synthetic construct
  source 1..20: mol_type = other RNA
actctcaagtccactgacag

SEQ ID NO: 4417 - RNA, 20 nt, synthetic construct
  source 1..20: mol_type = other RNA
ctgtcagtggacttgagagt

SEQ ID NO: 4418 - RNA, 20 nt, synthetic construct
  source 1..20: mol_type = other RNA
tgctttgaagcctctgtcag

SEQ ID NO: 4419 - RNA, 20 nt, synthetic construct
  source 1..20: mol_type = other RNA
atataatttccgtagaattt

SEQ ID NO: 4420 - RNA, 20 nt, synthetic construct
  source 1..20: mol_type = other RNA
taatttccgtagaattttgg

SEQ ID NO: 4421 - RNA, 20 nt, synthetic construct
  source 1..20: mol_type = other RNA
gtagaattttggaggcctgc

SEQ ID NO: 4422 - RNA, 20 nt, synthetic construct
  source 1..20: mol_type = other RNA
agcaggcctccaaaattcta

SEQ ID NO: 4423 - RNA, 20 nt, synthetic construct
  source 1..20: mol_type = other RNA
attttggaggcctgctggac

SEQ ID NO: 4424 - RNA, 20 nt, synthetic construct
  source 1..20: mol_type = other RNA
aggcctgctggactggcagc

SEQ ID NO: 4425 - RNA, 20 nt, synthetic construct
  source 1..20: mol_type = other RNA
gtaccagctgccagtccagc

SEQ ID NO: 4426 - RNA, 20 nt, synthetic construct
  source 1..20: mol_type = other RNA
ggtacacagctaaaagatag

SEQ ID NO: 4427 - RNA, 20 nt, synthetic construct
  source 1..20: mol_type = other RNA
gaggctagctaaaattgcac

SEQ ID NO: 4428 - RNA, 20 nt, synthetic construct
  source 1..20: mol_type = other RNA
aggctagctaaaattgcact

SEQ ID NO: 4429 - RNA, 20 nt, synthetic construct
  source 1..20: mol_type = other RNA
tagctaaaattgcactggga

SEQ ID NO: 4430 - RNA, 20 nt, synthetic construct
  source 1..20: mol_type = other RNA
tcagagggagaatgcagttc

SEQ ID NO: 4431 - RNA, 20 nt, synthetic construct
  source 1..20: mol_type = other RNA
gcattctccctctgaagtgg

SEQ ID NO: 4432 - RNA, 20 nt, synthetic construct
  source 1..20: mol_type = other RNA
ctccctctgaagtggaggaa

SEQ ID NO: 4433 - RNA, 20 nt, synthetic construct
  source 1..20: mol_type = other RNA
tgcctttcctccacttcaga

SEQ ID NO: 4434 - RNA, 20 nt, synthetic construct
  source 1..20: mol_type = other RNA
gtgcctttcctccacttcag

SEQ ID NO: 4435 - RNA, 20 nt, synthetic construct
  source 1..20: mol_type = other RNA
ggaggaaaggcaccttaatt

SEQ ID NO: 4436 - RNA, 20 nt, synthetic construct
  source 1..20: mol_type = other RNA
gaggaaaggcaccttaattt

SEQ ID NO: 4437 - RNA, 20 nt, synthetic construct
  source 1..20: mol_type = other RNA
acatctggcttcccaaatta

SEQ ID NO: 4438 - RNA, 20 nt, synthetic construct
  source 1..20: mol_type = other RNA
gccagatgtagaatttatga

SEQ ID NO: 4439 - RNA, 20 nt, synthetic construct
  source 1..20: mol_type = other RNA
ccagatgtagaatttatgat

SEQ ID NO: 4440 - RNA, 20 nt, synthetic construct
  source 1..20: mol_type = other RNA
cagatgtagaatttatgatg

SEQ ID NO: 4441 - RNA, 20 nt, synthetic construct
  source 1..20: mol_type = other RNA
cccatcataaattctacatc

SEQ ID NO: 4442 - RNA, 20 nt, synthetic construct
  source 1..20: mol_type = other RNA
tatgatggggatgtcgacca

SEQ ID NO: 4443 - RNA, 20 nt, synthetic construct
  source 1..20: mol_type = other RNA
tctcttgggcaggatgacct

SEQ ID NO: 4444 - RNA, 20 nt, synthetic construct
  source 1..20: mol_type = other RNA
ctgcccaagagatttcttcc

SEQ ID NO: 4445 - RNA, 20 nt, synthetic construct
  source 1..20: mol_type = other RNA
tgcccaagagatttcttcca

SEQ ID NO: 4446 - RNA, 20 nt, synthetic construct
  source 1..20: mol_type = other RNA
gcccaagagatttcttccag

SEQ ID NO: 4447 - RNA, 20 nt, synthetic construct
  source 1..20: mol_type = other RNA
cccaagagatttcttccagg

SEQ ID NO: 4448 - RNA, 20 nt, synthetic construct
  source 1..20: mol_type = other RNA
ctggaagaaatctcttgggc

SEQ ID NO: 4449 - RNA, 20 nt, synthetic construct
  source 1..20: mol_type = other RNA
ccccctggaagaaatctctt

SEQ ID NO: 4450 - RNA, 20 nt, synthetic construct
  source 1..20: mol_type = other RNA
accccctggaagaaatctct

SEQ ID NO: 4451 - RNA, 20 nt, synthetic construct
  source 1..20: mol_type = other RNA
atttcttccagggggtcaga

SEQ ID NO: 4452 - RNA, 20 nt, synthetic construct
  source 1..20: mol_type = other RNA
gggggtcagatggacccagc

SEQ ID NO: 4453 - RNA, 20 nt, synthetic construct
  source 1..20: mol_type = other RNA
ggggtcagatggacccagca

SEQ ID NO: 4454 - RNA, 20 nt, synthetic construct
  source 1..20: mol_type = other RNA
gctgggtccatctgaccccc

SEQ ID NO: 4455 - RNA, 20 nt, synthetic construct
  source 1..20: mol_type = other RNA
cagatggacccagcagggtc

SEQ ID NO: 4456 - RNA, 20 nt, synthetic construct
  source 1..20: mol_type = other RNA
gacccagcagggtctggatg

SEQ ID NO: 4457 - RNA, 20 nt, synthetic construct
  source 1..20: mol_type = other RNA
tgcctcatccagaccctgct

SEQ ID NO: 4458 - RNA, 20 nt, synthetic construct
  source 1..20: mol_type = other RNA
ctgcctcatccagaccctgc

SEQ ID NO: 4459 - RNA, 20 nt, synthetic construct
  source 1..20: mol_type = other RNA
atcagaagctgcgagcaatg

SEQ ID NO: 4460 - RNA, 20 nt, synthetic construct
  source 1..20: mol_type = other RNA
tcagaagctgcgagcaatgt

SEQ ID NO: 4461 - RNA, 20 nt, synthetic construct
  source 1..20: mol_type = other RNA
ctgcgagcaatgtgggagca

SEQ ID NO: 4462 - RNA, 20 nt, synthetic construct
  source 1..20: mol_type = other RNA
tgcgagcaatgtgggagcaa

SEQ ID NO: 4463 - RNA, 20 nt, synthetic construct
  source 1..20: mol_type = other RNA
agcaatgtgggagcaaggga

SEQ ID NO: 4464 - RNA, 20 nt, synthetic construct
  source 1..20: mol_type = other RNA
tgtgggagcaagggaaggca

SEQ ID NO: 4465 - RNA, 20 nt, synthetic construct
  source 1..20: mol_type = other RNA
aaggcaaggctgccagagta

SEQ ID NO: 4466 - RNA, 20 nt, synthetic construct
  source 1..20: mol_type = other RNA
gcaaggctgccagagtaagg

SEQ ID NO: 4467 - RNA, 20 nt, synthetic construct
  source 1..20: mol_type = other RNA
cagagtaaggtggctgcagt

SEQ ID NO: 4468 - RNA, 20 nt, synthetic construct
  source 1..20: mol_type = other RNA
agtaaggtggctgcagttgg

SEQ ID NO: 4469 - RNA, 20 nt, synthetic construct
  source 1..20: mol_type = other RNA
gtaaggtggctgcagttgga

SEQ ID NO: 4470 - RNA, 20 nt, synthetic construct
  source 1..20: mol_type = other RNA
taaggtggctgcagttggag

SEQ ID NO: 4471 - RNA, 20 nt, synthetic construct
  source 1..20: mol_type = other RNA
cagttggaggggcccagcag

SEQ ID NO: 4472 - RNA, 20 nt, synthetic construct
  source 1..20: mol_type = other RNA
gggcccagcagaggagcaca

SEQ ID NO: 4473 - RNA, 20 nt, synthetic construct
  source 1..20: mol_type = other RNA
actccgtgtgctcctctgct

SEQ ID NO: 4474 - RNA, 20 nt, synthetic construct
  source 1..20: mol_type = other RNA
cactccgtgtgctcctctgc

SEQ ID NO: 4475 - RNA, 20 nt, synthetic construct
  source 1..20: mol_type = other RNA
gagcacacggagtgcccatg

SEQ ID NO: 4476 - RNA, 20 nt, synthetic construct
  source 1..20: mol_type = other RNA
acacggagtgcccatgtgga

SEQ ID NO: 4477 - RNA, 20 nt, synthetic construct
  source 1..20: mol_type = other RNA
ttttaaagggccttccacat

SEQ ID NO: 4478 - RNA, 20 nt, synthetic construct
  source 1..20: mol_type = other RNA
gttttaaagggccttccaca

SEQ ID NO: 4479 - RNA, 20 nt, synthetic construct
  source 1..20: mol_type = other RNA
aggccctttaaaaccagctc

SEQ ID NO: 4480 - RNA, 20 nt, synthetic construct
  source 1..20: mol_type = other RNA
aagcctgagctggttttaaa

SEQ ID NO: 4481 - RNA, 20 nt, synthetic construct
  source 1..20: mol_type = other RNA
gaagcctgagctggttttaa

SEQ ID NO: 4482 - RNA, 20 nt, synthetic construct
  source 1..20: mol_type = other RNA
agctcaggcttccagaagta

SEQ ID NO: 4483 - RNA, 20 nt, synthetic construct
  source 1..20: mol_type = other RNA
atacttctggaagcctgagc

SEQ ID NO: 4484 - RNA, 20 nt, synthetic construct
  source 1..20: mol_type = other RNA
gtattagtctgccatacttc

SEQ ID NO: 4485 - RNA, 20 nt, synthetic construct
  source 1..20: mol_type = other RNA
ggttttcattcattcattac

SEQ ID NO: 4486 - RNA, 20 nt, synthetic construct
  source 1..20: mol_type = other RNA
accaattattattgttttgt

SEQ ID NO: 4487 - RNA, 20 nt, synthetic construct
  source 1..20: mol_type = other RNA
ccaattattattgttttgtt

SEQ ID NO: 4488 - RNA, 20 nt, synthetic construct
  source 1..20: mol_type = other RNA
cccaacaaaacaataataat

SEQ ID NO: 4489 - RNA, 20 nt, synthetic construct
  source 1..20: mol_type = other RNA
tattgttttgttgggttcag

SEQ ID NO: 4490 - RNA, 20 nt, synthetic construct
  source 1..20: mol_type = other RNA
aatgaaaaaaaaatgtctac

SEQ ID NO: 4491 - RNA, 20 nt, synthetic construct
  source 1..20: mol_type = other RNA
atgaaaaaaaaatgtctaca

SEQ ID NO: 4492 - RNA, 20 nt, synthetic construct
  source 1..20: mol_type = other RNA
tgaaaaaaaaatgtctacag

SEQ ID NO: 4493 - RNA, 20 nt, synthetic construct
  source 1..20: mol_type = other RNA
aaatgtctacaggggcaaaa

SEQ ID NO: 4494 - RNA, 20 nt, synthetic construct
  source 1..20: mol_type = other RNA
ctacaggggcaaaaaggaaa

SEQ ID NO: 4495 - RNA, 20 nt, synthetic construct
  source 1..20: mol_type = other RNA
cagtaacaaccaaaaatccc

SEQ ID NO: 4496 - RNA, 20 nt, synthetic construct
  source 1..20: mol_type = other RNA
agtaacaaccaaaaatccct

SEQ ID NO: 4497 - RNA, 20 nt, synthetic construct
  source 1..20: mol_type = other RNA
gctcactgcccagggatttt

SEQ ID NO: 4498 - RNA, 20 nt, synthetic construct
  source 1..20: mol_type = other RNA
tgggcagtgagcctcagaaa

SEQ ID NO: 4499 - RNA, 20 nt, synthetic construct
  source 1..20: mol_type = other RNA
gggcagtgagcctcagaaaa

SEQ ID NO: 4500 - RNA, 20 nt, synthetic construct
  source 1..20: mol_type = other RNA
tttctgaggctcactgccca

SEQ ID NO: 4501 - RNA, 20 nt, synthetic construct
  source 1..20: mol_type = other RNA
ttttctgaggctcactgccc

SEQ ID NO: 4502 - RNA, 20 nt, synthetic construct
  source 1..20: mol_type = other RNA
tgagcctcagaaaaggggaa

SEQ ID NO: 4503 - RNA, 20 nt, synthetic construct
  source 1..20: mol_type = other RNA
aggaccgttccccttttctg

SEQ ID NO: 4504 - RNA, 20 nt, synthetic construct
  source 1..20: mol_type = other RNA
aaaaggggaacggtcctgtg

SEQ ID NO: 4505 - RNA, 20 nt, synthetic construct
  source 1..20: mol_type = other RNA
aacggtcctgtgaggacatg

SEQ ID NO: 4506 - RNA, 20 nt, synthetic construct
  source 1..20: mol_type = other RNA
agatcaccacatgtcctcac

SEQ ID NO: 4507 - RNA, 20 nt, synthetic construct
  source 1..20: mol_type = other RNA
tggtgatctcacgtgatctc

SEQ ID NO: 4508 - RNA, 20 nt, synthetic construct
  source 1..20: mol_type = other RNA
ggtgatctcacgtgatctct

SEQ ID NO: 4509 - RNA, 20 nt, synthetic construct
  source 1..20: mol_type = other RNA
gatctcacgtgatctctggg

SEQ ID NO: 4510 - RNA, 20 nt, synthetic construct
  source 1..20: mol_type = other RNA
tcacgtgatctctgggaggc

SEQ ID NO: 4511 - RNA, 20 nt, synthetic construct
  source 1..20: mol_type = other RNA
cacgtgatctctgggaggct

SEQ ID NO: 4512 - RNA, 20 nt, synthetic construct
  source 1..20: mol_type = other RNA
gaggctgggcctcagctctg

SEQ ID NO: 4513 - RNA, 20 nt, synthetic construct
  source 1..20: mol_type = other RNA
ctgggcctcagctctgtggc

SEQ ID NO: 4514 - RNA, 20 nt, synthetic construct
  source 1..20: mol_type = other RNA
tgggcctcagctctgtggct

SEQ ID NO: 4515 - RNA, 20 nt, synthetic construct
  source 1..20: mol_type = other RNA
gcctcagctctgtggctggg

SEQ ID NO: 4516 - RNA, 20 nt, synthetic construct
  source 1..20: mol_type = other RNA
cctcagctctgtggctgggt

SEQ ID NO: 4517 - RNA, 20 nt, synthetic construct
  source 1..20: mol_type = other RNA
ctcagctctgtggctgggtg

SEQ ID NO: 4518 - RNA, 20 nt, synthetic construct
  source 1..20: mol_type = other RNA
tcagctctgtggctgggtgg

SEQ ID NO: 4519 - RNA, 20 nt, synthetic construct
  source 1..20: mol_type = other RNA
cccacccagccacagagctg

SEQ ID NO: 4520 - RNA, 20 nt, synthetic construct
  source 1..20: mol_type = other RNA
ggggaactaaactaaaattc

SEQ ID NO: 4521 - RNA, 20 nt, synthetic construct
  source 1..20: mol_type = other RNA
gggaactaaactaaaattcc

SEQ ID NO: 4522 - RNA, 20 nt, synthetic construct
  source 1..20: mol_type = other RNA
ggaactaaactaaaattccg

SEQ ID NO: 4523 - RNA, 20 nt, synthetic construct
  source 1..20: mol_type = other RNA
actaaaattccggggttaca

SEQ ID NO: 4524 - RNA, 20 nt, synthetic construct
  source 1..20: mol_type = other RNA
cggggttacatggcagcatc

SEQ ID NO: 4525 - RNA, 20 nt, synthetic construct
  source 1..20: mol_type = other RNA
cagatgctgccatgtaaccc

SEQ ID NO: 4526 - RNA, 20 nt, synthetic construct
  source 1..20: mol_type = other RNA
tggcagcatctggaaggcaa

SEQ ID NO: 4527 - RNA, 20 nt, synthetic construct
  source 1..20: mol_type = other RNA
gaaggcaatggaattgtctc

SEQ ID NO: 4528 - RNA, 20 nt, synthetic construct
  source 1..20: mol_type = other RNA
caggaccgcagtacccccgc

SEQ ID NO: 4529 - RNA, 20 nt, synthetic construct
  source 1..20: mol_type = other RNA
gctgtcctgcgggggtactg

SEQ ID NO: 4530 - RNA, 20 nt, synthetic construct
  source 1..20: mol_type = other RNA
agggtgctgctgtcctgcgg

SEQ ID NO: 4531 - RNA, 20 nt, synthetic construct
  source 1..20: mol_type = other RNA
tagggtgctgctgtcctgcg

SEQ ID NO: 4532 - RNA, 20 nt, synthetic construct
  source 1..20: mol_type = other RNA
atagggtgctgctgtcctgc

SEQ ID NO: 4533 - RNA, 20 nt, synthetic construct
  source 1..20: mol_type = other RNA
catagggtgctgctgtcctg

SEQ ID NO: 4534 - RNA, 20 nt, synthetic construct
  source 1..20: mol_type = other RNA
cagcagcaccctatgactac

SEQ ID NO: 4535 - RNA, 20 nt, synthetic construct
  source 1..20: mol_type = other RNA
tgcttttgccagtagtcata

SEQ ID NO: 4536 - RNA, 20 nt, synthetic construct
  source 1..20: mol_type = other RNA
ttgcttttgccagtagtcat

SEQ ID NO: 4537 - RNA, 20 nt, synthetic construct
  source 1..20: mol_type = other RNA
gagaaaagcatccttgactt

SEQ ID NO: 4538 - RNA, 20 nt, synthetic construct
  source 1..20: mol_type = other RNA
aagtcttggggcctaagtca

SEQ ID NO: 4539 - RNA, 20 nt, synthetic construct
  source 1..20: mol_type = other RNA
ccaagactttttctacaatt

SEQ ID NO: 4540 - RNA, 20 nt, synthetic construct
  source 1..20: mol_type = other RNA
taattgtagaaaaagtcttg

SEQ ID NO: 4541 - RNA, 20 nt, synthetic construct
  source 1..20: mol_type = other RNA
ctaattgtagaaaaagtctt

SEQ ID NO: 4542 - RNA, 20 nt, synthetic construct
  source 1..20: mol_type = other RNA
cctaattgtagaaaaagtct

SEQ ID NO: 4543 - RNA, 20 nt, synthetic construct
  source 1..20: mol_type = other RNA
caaatatgagctagcaatta

SEQ ID NO: 4544 - RNA, 20 nt, synthetic construct
  source 1..20: mol_type = other RNA
cttaattgctagctcatatt

SEQ ID NO: 4545 - RNA, 20 nt, synthetic construct
  source 1..20: mol_type = other RNA
ttaaggtttactaaacagac

SEQ ID NO: 4546 - RNA, 20 nt, synthetic construct
  source 1..20: mol_type = other RNA
taaggtttactaaacagaca

SEQ ID NO: 4547 - RNA, 20 nt, synthetic construct
  source 1..20: mol_type = other RNA
agacagggaaacgaaacatc

SEQ ID NO: 4548 - RNA, 20 nt, synthetic construct
  source 1..20: mol_type = other RNA
agaacagatgcaaagtgcca

SEQ ID NO: 4549 - RNA, 20 nt, synthetic construct
  source 1..20: mol_type = other RNA
actgaagcatctgaagtcct

SEQ ID NO: 4550 - RNA, 20 nt, synthetic construct
  source 1..20: mol_type = other RNA
gttattttatagtcagtatt

SEQ ID NO: 4551 - RNA, 20 nt, synthetic construct
  source 1..20: mol_type = other RNA
ataaaataactacatatgaa

SEQ ID NO: 4552 - RNA, 20 nt, synthetic construct
  source 1..20: mol_type = other RNA
agtgactatcaaaaatgacc

SEQ ID NO: 4553 - RNA, 20 nt, synthetic construct
  source 1..20: mol_type = other RNA
actatcaaaaatgaccaggc

SEQ ID NO: 4554 - RNA, 20 nt, synthetic construct
  source 1..20: mol_type = other RNA
ctatcaaaaatgaccaggca

SEQ ID NO: 4555 - RNA, 20 nt, synthetic construct
  source 1..20: mol_type = other RNA
caaaaatgaccaggcagggc

SEQ ID NO: 4556 - RNA, 20 nt, synthetic construct
  source 1..20: mol_type = other RNA
aaaaatgaccaggcagggct

SEQ ID NO: 4557 - RNA, 20 nt, synthetic construct
  source 1..20: mol_type = other RNA
ccaggcagggctgggtgcag

SEQ ID NO: 4558 - RNA, 20 nt, synthetic construct
  source 1..20: mol_type = other RNA
ccactgcacccagccctgcc

SEQ ID NO: 4559 - RNA, 20 nt, synthetic construct
  source 1..20: mol_type = other RNA
cgaccgtaatcccaccactt

SEQ ID NO: 4560 - RNA, 20 nt, synthetic construct
  source 1..20: mol_type = other RNA
gaccgtaatcccaccacttt

SEQ ID NO: 4561 - RNA, 20 nt, synthetic construct
  source 1..20: mol_type = other RNA
cgtaatcccaccactttggg

SEQ ID NO: 4562 - RNA, 20 nt, synthetic construct
  source 1..20: mol_type = other RNA
ctcccaaagtggtgggatta

SEQ ID NO: 4563 - RNA, 20 nt, synthetic construct
  source 1..20: mol_type = other RNA
cccaccactttgggaggcca

SEQ ID NO: 4564 - RNA, 20 nt, synthetic construct
  source 1..20: mol_type = other RNA
accactttgggaggccaagg

SEQ ID NO: 4565 - RNA, 20 nt, synthetic construct
  source 1..20: mol_type = other RNA
ccactttgggaggccaaggc

SEQ ID NO: 4566 - RNA, 20 nt, synthetic construct
  source 1..20: mol_type = other RNA
ccttggcctcccaaagtggt

SEQ ID NO: 4567 - RNA, 20 nt, synthetic construct
  source 1..20: mol_type = other RNA
gccttggcctcccaaagtgg

SEQ ID NO: 4568 - RNA, 20 nt, synthetic construct
  source 1..20: mol_type = other RNA
ctttgggaggccaaggcggg

SEQ ID NO: 4569 - RNA, 20 nt, synthetic construct
  source 1..20: mol_type = other RNA
cccgccttggcctcccaaag

SEQ ID NO: 4570 - RNA, 20 nt, synthetic construct
  source 1..20: mol_type = other RNA
ctcaggtgatccacccgcct

SEQ ID NO: 4571 - RNA, 20 nt, synthetic construct
  source 1..20: mol_type = other RNA
cgggtggatcacctgagtcc

SEQ ID NO: 4572 - RNA, 20 nt, synthetic construct
  source 1..20: mol_type = other RNA
tcacctgagtccaggagttc

SEQ ID NO: 4573 - RNA, 20 nt, synthetic construct
  source 1..20: mol_type = other RNA
ggtcctgaactcctggactc

SEQ ID NO: 4574 - RNA, 20 nt, synthetic construct
  source 1..20: mol_type = other RNA
ccaggagttcaggaccagcc

SEQ ID NO: 4575 - RNA, 20 nt, synthetic construct
  source 1..20: mol_type = other RNA
ccaggctggtcctgaactcc

SEQ ID NO: 4576 - RNA, 20 nt, synthetic construct
  source 1..20: mol_type = other RNA
caggaccagcctggccaaca

SEQ ID NO: 4577 - RNA, 20 nt, synthetic construct
  source 1..20: mol_type = other RNA
tttcaccatgttggccaggc

SEQ ID NO: 4578 - RNA, 20 nt, synthetic construct
  source 1..20: mol_type = other RNA
ggggtttcaccatgttggcc

SEQ ID NO: 4579 - RNA, 20 nt, synthetic construct
  source 1..20: mol_type = other RNA
gagacggggtttcaccatgt

SEQ ID NO: 4580 - RNA, 20 nt, synthetic construct
  source 1..20: mol_type = other RNA
ttgtatttttagtagagacg

SEQ ID NO: 4581 - RNA, 20 nt, synthetic construct
  source 1..20: mol_type = other RNA
tttgtatttttagtagagac

SEQ ID NO: 4582 - RNA, 20 nt, synthetic construct
  source 1..20: mol_type = other RNA
ttttgtatttttagtagaga

SEQ ID NO: 4583 - RNA, 20 nt, synthetic construct
  source 1..20: mol_type = other RNA
taaaaatacaaaaattagcc

SEQ ID NO: 4584 - RNA, 20 nt, synthetic construct
  source 1..20: mol_type = other RNA
atacaaaaattagccaggcg

SEQ ID NO: 4585 - RNA, 20 nt, synthetic construct
  source 1..20: mol_type = other RNA
caaaaattagccaggcgtgg

SEQ ID NO: 4586 - RNA, 20 nt, synthetic construct
  source 1..20: mol_type = other RNA
caggcaagtgccaccacgcc

SEQ ID NO: 4587 - RNA, 20 nt, synthetic construct
  source 1..20: mol_type = other RNA
tggcacttgcctgtaatccc

SEQ ID NO: 4588 - RNA, 20 nt, synthetic construct
  source 1..20: mol_type = other RNA
tgcctgtaatcccaggtact

SEQ ID NO: 4589 - RNA, 20 nt, synthetic construct
  source 1..20: mol_type = other RNA
gcctgtaatcccaggtactc

SEQ ID NO: 4590 - RNA, 20 nt, synthetic construct
  source 1..20: mol_type = other RNA
tgtaatcccaggtactcggg

SEQ ID NO: 4591 - RNA, 20 nt, synthetic construct
  source 1..20: mol_type = other RNA
tcccgagtacctgggattac

SEQ ID NO: 4592 - RNA, 20 nt, synthetic construct
  source 1..20: mol_type = other RNA
cccaggtactcgggaggctg

SEQ ID NO: 4593 - RNA, 20 nt, synthetic construct
  source 1..20: mol_type = other RNA
ggtactcgggaggctgaggc

SEQ ID NO: 4594 - RNA, 20 nt, synthetic construct
  source 1..20: mol_type = other RNA
cctcagcctcccgagtacct

SEQ ID NO: 4595 - RNA, 20 nt, synthetic construct
  source 1..20: mol_type = other RNA
gcctcagcctcccgagtacc

SEQ ID NO: 4596 - RNA, 20 nt, synthetic construct
  source 1..20: mol_type = other RNA
gcaggagaatcacttgaacc

SEQ ID NO: 4597 - RNA, 20 nt, synthetic construct
  source 1..20: mol_type = other RNA
caggagaatcacttgaacct

SEQ ID NO: 4598 - RNA, 20 nt, synthetic construct
  source 1..20: mol_type = other RNA
gagaatcacttgaacctggg

SEQ ID NO: 4599 - RNA, 20 nt, synthetic construct
  source 1..20: mol_type = other RNA
aatcacttgaacctgggagg

SEQ ID NO: 4600 - RNA, 20 nt, synthetic construct
  source 1..20: mol_type = other RNA
cacttgaacctgggaggcgg

SEQ ID NO: 4601 - RNA, 20 nt, synthetic construct
  source 1..20: mol_type = other RNA
tactgaaacctccgcctccc

SEQ ID NO: 4602 - RNA, 20 nt, synthetic construct
  source 1..20: mol_type = other RNA
ggaatgcagtggcgcgatct

SEQ ID NO: 4603 - RNA, 20 nt, synthetic construct
  source 1..20: mol_type = other RNA
cgcgccactgcattccagcc

SEQ ID NO: 4604 - RNA, 20 nt, synthetic construct
  source 1..20: mol_type = other RNA
gcgccactgcattccagcct

SEQ ID NO: 4605 - RNA, 20 nt, synthetic construct
  source 1..20: mol_type = other RNA
ttgcccaggctggaatgcag

SEQ ID NO: 4606 - RNA, 20 nt, synthetic construct
  source 1..20: mol_type = other RNA
tcgctcattgttgcccaggc

SEQ ID NO: 4607 - RNA, 20 nt, synthetic construct
  source 1..20: mol_type = other RNA
agtttcgctcattgttgccc

SEQ ID NO: 4608 - RNA, 20 nt, synthetic construct
  source 1..20: mol_type = other RNA
ttttttttttttttttgaga

SEQ ID NO: 4609 - RNA, 20 nt, synthetic construct
  source 1..20: mol_type = other RNA
aaaaaaaaaaaaaaatgacc

SEQ ID NO: 4610 - RNA, 20 nt, synthetic construct
  source 1..20: mol_type = other RNA
tttgcaaagctgaaactgcc

SEQ ID NO: 4611 - RNA, 20 nt, synthetic construct
  source 1..20: mol_type = other RNA
ttgcaaactgaaaagagctg

SEQ ID NO: 4612 - RNA, 20 nt, synthetic construct
  source 1..20: mol_type = other RNA
ctgaaaagagctgtggagat

SEQ ID NO: 4613 - RNA, 20 nt, synthetic construct
  source 1..20: mol_type = other RNA
acacttaaaaatagcgaaga

SEQ ID NO: 4614 - RNA, 20 nt, synthetic construct
  source 1..20: mol_type = other RNA
ccacaattttttaaatgaca

SEQ ID NO: 4615 - RNA, 20 nt, synthetic construct
  source 1..20: mol_type = other RNA
ccttgtcatttaaaaaattg

SEQ ID NO: 4616 - RNA, 20 nt, synthetic construct
  source 1..20: mol_type = other RNA
taaaaatagaattagtgaat

SEQ ID NO: 4617 - RNA, 20 nt, synthetic construct
  source 1..20: mol_type = other RNA
aatagaattagtgaattgga

SEQ ID NO: 4618 - RNA, 20 nt, synthetic construct
  source 1..20: mol_type = other RNA
aaatgaaaaaattacctaaa

SEQ ID NO: 4619 - RNA, 20 nt, synthetic construct
  source 1..20: mol_type = other RNA
aaaggcaatacagtaagaca

SEQ ID NO: 4620 - RNA, 20 nt, synthetic construct
  source 1..20: mol_type = other RNA
gtcttactgtattgcctttt

SEQ ID NO: 4621 - RNA, 20 nt, synthetic construct
  source 1..20: mol_type = other RNA
taaagaaatgttaacctaaa

SEQ ID NO: 4622 - RNA, 20 nt, synthetic construct
  source 1..20: mol_type = other RNA
aaatggagaatacaatgaga

SEQ ID NO: 4623 - RNA, 20 nt, synthetic construct
  source 1..20: mol_type = other RNA
tctcattgtattctccattt

SEQ ID NO: 4624 - RNA, 20 nt, synthetic construct
  source 1..20: mol_type = other RNA
aggtccaaaatatgtctcat

SEQ ID NO: 4625 - RNA, 20 nt, synthetic construct
  source 1..20: mol_type = other RNA
gtctccgatgagacatattt

SEQ ID NO: 4626 - RNA, 20 nt, synthetic construct
  source 1..20: mol_type = other RNA
cctagaagaaaagaatagaa

SEQ ID NO: 4627 - RNA, 20 nt, synthetic construct
  source 1..20: mol_type = other RNA
gaagaaaagaatagaaagga

SEQ ID NO: 4628 - RNA, 20 nt, synthetic construct
  source 1..20: mol_type = other RNA
cctttctattcttttcttct

SEQ ID NO: 4629 - RNA, 20 nt, synthetic construct
  source 1..20: mol_type = other RNA
gaaaagaatagaaaggaagg

SEQ ID NO: 4630 - RNA, 20 nt, synthetic construct
  source 1..20: mol_type = other RNA
gaatagaaaggaaggaggaa

SEQ ID NO: 4631 - RNA, 20 nt, synthetic construct
  source 1..20: mol_type = other RNA
aatagaaaggaaggaggaaa

SEQ ID NO: 4632 - RNA, 20 nt, synthetic construct
  source 1..20: mol_type = other RNA
aggaggaaagggaatattta

SEQ ID NO: 4633 - RNA, 20 nt, synthetic construct
  source 1..20: mol_type = other RNA
atgataactgagatgtttcc

SEQ ID NO: 4634 - RNA, 20 nt, synthetic construct
  source 1..20: mol_type = other RNA
tttatgtcttttaacactcc

SEQ ID NO: 4635 - RNA, 20 nt, synthetic construct
  source 1..20: mol_type = other RNA
aatccacagatatactaatc

SEQ ID NO: 4636 - RNA, 20 nt, synthetic construct
  source 1..20: mol_type = other RNA
atccacagatatactaatca

SEQ ID NO: 4637 - RNA, 20 nt, synthetic construct
  source 1..20: mol_type = other RNA
taccctgattagtatatctg

SEQ ID NO: 4638 - RNA, 20 nt, synthetic construct
  source 1..20: mol_type = other RNA
gggtaaatgaaaagaaattc

SEQ ID NO: 4639 - RNA, 20 nt, synthetic construct
  source 1..20: mol_type = other RNA
aaatgaaaagaaattcaggc

SEQ ID NO: 4640 - RNA, 20 nt, synthetic construct
  source 1..20: mol_type = other RNA
aatgaaaagaaattcaggct

SEQ ID NO: 4641 - RNA, 20 nt, synthetic construct
  source 1..20: mol_type = other RNA
aaagaaattcaggctgggcg

SEQ ID NO: 4642 - RNA, 20 nt, synthetic construct
  source 1..20: mol_type = other RNA
gaaattcaggctgggcgcgg

SEQ ID NO: 4643 - RNA, 20 nt, synthetic construct
  source 1..20: mol_type = other RNA
caccttaaaccccagaactt

SEQ ID NO: 4644 - RNA, 20 nt, synthetic construct
  source 1..20: mol_type = other RNA
accttaaaccccagaacttt

SEQ ID NO: 4645 - RNA, 20 nt, synthetic construct
  source 1..20: mol_type = other RNA
ttaaaccccagaactttggg

SEQ ID NO: 4646 - RNA, 20 nt, synthetic construct
  source 1..20: mol_type = other RNA
tcccaaagttctggggttta

SEQ ID NO: 4647 - RNA, 20 nt, synthetic construct
  source 1..20: mol_type = other RNA
cccagaactttgggaggctg

SEQ ID NO: 4648 - RNA, 20 nt, synthetic construct
  source 1..20: mol_type = other RNA
agaactttgggaggctgagg

SEQ ID NO: 4649 - RNA, 20 nt, synthetic construct
  source 1..20: mol_type = other RNA
ctcagcctcccaaagttctg

SEQ ID NO: 4650 - RNA, 20 nt, synthetic construct
  source 1..20: mol_type = other RNA
cctcagcctcccaaagttct

SEQ ID NO: 4651 - RNA, 20 nt, synthetic construct
  source 1..20: mol_type = other RNA
gcctcagcctcccaaagttc

SEQ ID NO: 4652 - RNA, 20 nt, synthetic construct
  source 1..20: mol_type = other RNA
ctttgggaggctgaggcggg

SEQ ID NO: 4653 - RNA, 20 nt, synthetic construct
  source 1..20: mol_type = other RNA
tgaggcgggtggatcacctg

SEQ ID NO: 4654 - RNA, 20 nt, synthetic construct
  source 1..20: mol_type = other RNA
cgggtggatcacctgaggtc

SEQ ID NO: 4655 - RNA, 20 nt, synthetic construct
  source 1..20: mol_type = other RNA
ggtcttgaactcctgacctc

SEQ ID NO: 4656 - RNA, 20 nt, synthetic construct
  source 1..20: mol_type = other RNA
caagaccatcctgaccaaca

SEQ ID NO: 4657 - RNA, 20 nt, synthetic construct
  source 1..20: mol_type = other RNA
tttctccatgttggtcagga

SEQ ID NO: 4658 - RNA, 20 nt, synthetic construct
  source 1..20: mol_type = other RNA
ggggtttctccatgttggtc

SEQ ID NO: 4659 - RNA, 20 nt, synthetic construct
  source 1..20: mol_type = other RNA
gatatggggtttctccatgt

SEQ ID NO: 4660 - RNA, 20 nt, synthetic construct
  source 1..20: mol_type = other RNA
ttgtatttttagtagatatg

SEQ ID NO: 4661 - RNA, 20 nt, synthetic construct
  source 1..20: mol_type = other RNA
tttgtatttttagtagatat

SEQ ID NO: 4662 - RNA, 20 nt, synthetic construct
  source 1..20: mol_type = other RNA
gtttgtatttttagtagata

SEQ ID NO: 4663 - RNA, 20 nt, synthetic construct
  source 1..20: mol_type = other RNA
actaaaaatacaaacttagc

SEQ ID NO: 4664 - RNA, 20 nt, synthetic construct
  source 1..20: mol_type = other RNA
ctaaaaatacaaacttagcc

SEQ ID NO: 4665 - RNA, 20 nt, synthetic construct
  source 1..20: mol_type = other RNA
aatacaaacttagccgggca

SEQ ID NO: 4666 - RNA, 20 nt, synthetic construct
  source 1..20: mol_type = other RNA
acaaacttagccgggcatgg

SEQ ID NO: 4667 - RNA, 20 nt, synthetic construct
  source 1..20: mol_type = other RNA
caggtgcatgccaccatgcc

SEQ ID NO: 4668 - RNA, 20 nt, synthetic construct
  source 1..20: mol_type = other RNA
cacctgtaatcccagctact

SEQ ID NO: 4669 - RNA, 20 nt, synthetic construct
  source 1..20: mol_type = other RNA
acctgtaatcccagctactc

SEQ ID NO: 4670 - RNA, 20 nt, synthetic construct
  source 1..20: mol_type = other RNA
tgtaatcccagctactcggg

SEQ ID NO: 4671 - RNA, 20 nt, synthetic construct
  source 1..20: mol_type = other RNA
tcccgagtagctgggattac

SEQ ID NO: 4672 - RNA, 20 nt, synthetic construct
  source 1..20: mol_type = other RNA
cccagctactcgggaggctg

SEQ ID NO: 4673 - RNA, 20 nt, synthetic construct
  source 1..20: mol_type = other RNA
cctcagcctcccgagtagct

SEQ ID NO: 4674 - RNA, 20 nt, synthetic construct
  source 1..20: mol_type = other RNA
gcctcagcctcccgagtagc

SEQ ID NO: 4675 - RNA, 20 nt, synthetic construct
  source 1..20: mol_type = other RNA
gcagaagaatcacttgaacc

SEQ ID NO: 4676 - RNA, 20 nt, synthetic construct
  source 1..20: mol_type = other RNA
cagaagaatcacttgaaccc

SEQ ID NO: 4677 - RNA, 20 nt, synthetic construct
  source 1..20: mol_type = other RNA
aagaatcacttgaacccggg

SEQ ID NO: 4678 - RNA, 20 nt, synthetic construct
  source 1..20: mol_type = other RNA
aatcacttgaacccgggagg

SEQ ID NO: 4679 - RNA, 20 nt, synthetic construct
  source 1..20: mol_type = other RNA
cacttgaacccgggaggcgg

SEQ ID NO: 4680 - RNA, 20 nt, synthetic construct
  source 1..20: mol_type = other RNA
cactgcaacctccgcctccc

SEQ ID NO: 4681 - RNA, 20 nt, synthetic construct
  source 1..20: mol_type = other RNA
tcactgcaacctccgcctcc

SEQ ID NO: 4682 - RNA, 20 nt, synthetic construct
  source 1..20: mol_type = other RNA
ggagtgcagtggcacgatct

SEQ ID NO: 4683 - RNA, 20 nt, synthetic construct
  source 1..20: mol_type = other RNA
cgtgccactgcactccagcc

SEQ ID NO: 4684 - RNA, 20 nt, synthetic construct
  source 1..20: mol_type = other RNA
gtgccactgcactccagcct

SEQ ID NO: 4685 - RNA, 20 nt, synthetic construct
  source 1..20: mol_type = other RNA
ttgcccaggctggagtgcag

SEQ ID NO: 4686 - RNA, 20 nt, synthetic construct
  source 1..20: mol_type = other RNA
tttgttcttgttgcccaggc

SEQ ID NO: 4687 - RNA, 20 nt, synthetic construct
  source 1..20: mol_type = other RNA
gagttttgttcttgttgccc

SEQ ID NO: 4688 - RNA, 20 nt, synthetic construct
  source 1..20: mol_type = other RNA
cttttcttttttttttgaga

SEQ ID NO: 4689 - RNA, 20 nt, synthetic construct
  source 1..20: mol_type = other RNA
aaagaaaagaaattcaatct

SEQ ID NO: 4690 - RNA, 20 nt, synthetic construct
  source 1..20: mol_type = other RNA
agagatgttaaattgcaaca

SEQ ID NO: 4691 - RNA, 20 nt, synthetic construct
  source 1..20: mol_type = other RNA
atgctggctttgtgttttct

SEQ ID NO: 4692 - RNA, 20 nt, synthetic construct
  source 1..20: mol_type = other RNA
tatgctggctttgtgttttc

SEQ ID NO: 4693 - RNA, 20 nt, synthetic construct
  source 1..20: mol_type = other RNA
cactgggtctggtcatatgc

SEQ ID NO: 4694 - RNA, 20 nt, synthetic construct
  source 1..20: mol_type = other RNA
aagggatttctcactgggtc

SEQ ID NO: 4695 - RNA, 20 nt, synthetic construct
  source 1..20: mol_type = other RNA
aatagaagggatttctcact

SEQ ID NO: 4696 - RNA, 20 nt, synthetic construct
  source 1..20: mol_type = other RNA
aaatagaagggatttctcac

SEQ ID NO: 4697 - RNA, 20 nt, synthetic construct
  source 1..20: mol_type = other RNA
ggtgatagtaagaaatagaa

SEQ ID NO: 4698 - RNA, 20 nt, synthetic construct
  source 1..20: mol_type = other RNA
aggtgatagtaagaaataga

SEQ ID NO: 4699 - RNA, 20 nt, synthetic construct
  source 1..20: mol_type = other RNA
aaaaggagtagaggaggggt

SEQ ID NO: 4700 - RNA, 20 nt, synthetic construct
  source 1..20: mol_type = other RNA
ggagaaaaggagtagaggag

SEQ ID NO: 4701 - RNA, 20 nt, synthetic construct
  source 1..20: mol_type = other RNA
gggagaaaaggagtagagga

SEQ ID NO: 4702 - RNA, 20 nt, synthetic construct
  source 1..20: mol_type = other RNA
ggggagaaaaggagtagagg

SEQ ID NO: 4703 - RNA, 20 nt, synthetic construct
  source 1..20: mol_type = other RNA
gctggggagaaaaggagtag

SEQ ID NO: 4704 - RNA, 20 nt, synthetic construct
  source 1..20: mol_type = other RNA
gagtgaatgctggggagaaa

SEQ ID NO: 4705 - RNA, 20 nt, synthetic construct
  source 1..20: mol_type = other RNA
ttctcattgagtgaatgctg

SEQ ID NO: 4706 - RNA, 20 nt, synthetic construct
  source 1..20: mol_type = other RNA
tttctcattgagtgaatgct

SEQ ID NO: 4707 - RNA, 20 nt, synthetic construct
  source 1..20: mol_type = other RNA
ctttctcattgagtgaatgc

SEQ ID NO: 4708 - RNA, 20 nt, synthetic construct
  source 1..20: mol_type = other RNA
actcaatgagaaagagtagc

SEQ ID NO: 4709 - RNA, 20 nt, synthetic construct
  source 1..20: mol_type = other RNA
atgagaaagagtagctggag

SEQ ID NO: 4710 - RNA, 20 nt, synthetic construct
  source 1..20: mol_type = other RNA
tgagaaagagtagctggagc

SEQ ID NO: 4711 - RNA, 20 nt, synthetic construct
  source 1..20: mol_type = other RNA
gaaagagtagctggagcggg

SEQ ID NO: 4712 - RNA, 20 nt, synthetic construct
  source 1..20: mol_type = other RNA
aaagagtagctggagcgggt

SEQ ID NO: 4713 - RNA, 20 nt, synthetic construct
  source 1..20: mol_type = other RNA
aagagtagctggagcgggtg

SEQ ID NO: 4714 - RNA, 20 nt, synthetic construct
  source 1..20: mol_type = other RNA
ctacctcctcccacataatc

SEQ ID NO: 4715 - RNA, 20 nt, synthetic construct
  source 1..20: mol_type = other RNA
cagattatgtgggaggaggt

SEQ ID NO: 4716 - RNA, 20 nt, synthetic construct
  source 1..20: mol_type = other RNA
catccagattatgtgggagg

SEQ ID NO: 4717 - RNA, 20 nt, synthetic construct
  source 1..20: mol_type = other RNA
atccatccagattatgtggg

SEQ ID NO: 4718 - RNA, 20 nt, synthetic construct
  source 1..20: mol_type = other RNA
ggcatccatccagattatgt

SEQ ID NO: 4719 - RNA, 20 nt, synthetic construct
  source 1..20: mol_type = other RNA
aggcatccatccagattatg

SEQ ID NO: 4720 - RNA, 20 nt, synthetic construct
  source 1..20: mol_type = other RNA
gcctacagccatgtcttcaa

SEQ ID NO: 4721 - RNA, 20 nt, synthetic construct
  source 1..20: mol_type = other RNA
cctacagccatgtcttcaat

SEQ ID NO: 4722 - RNA, 20 nt, synthetic construct
  source 1..20: mol_type = other RNA
cccattgaagacatggctgt

SEQ ID NO: 4723 - RNA, 20 nt, synthetic construct
  source 1..20: mol_type = other RNA
ttccttgcccattgaagaca

SEQ ID NO: 4724 - RNA, 20 nt, synthetic construct
  source 1..20: mol_type = other RNA
gaattgctactaaattaaga

SEQ ID NO: 4725 - RNA, 20 nt, synthetic construct
  source 1..20: mol_type = other RNA
ttaacacaactgtccaatgt

SEQ ID NO: 4726 - RNA, 20 nt, synthetic construct
  source 1..20: mol_type = other RNA
gtctctctttcttcctacat

SEQ ID NO: 4727 - RNA, 20 nt, synthetic construct
  source 1..20: mol_type = other RNA
cacaagctttttgttgagga

SEQ ID NO: 4728 - RNA, 20 nt, synthetic construct
  source 1..20: mol_type = other RNA
ttatcacaagctttttgttg

SEQ ID NO: 4729 - RNA, 20 nt, synthetic construct
  source 1..20: mol_type = other RNA
acttgcaatgcataggtaac

SEQ ID NO: 4730 - RNA, 20 nt, synthetic construct
  source 1..20: mol_type = other RNA
ttctgcaacttgcaatgcat

SEQ ID NO: 4731 - RNA, 20 nt, synthetic construct
  source 1..20: mol_type = other RNA
caaatggtgagagatagact

SEQ ID NO: 4732 - RNA, 20 nt, synthetic construct
  source 1..20: mol_type = other RNA
ctctcaccatttgctttccc

SEQ ID NO: 4733 - RNA, 20 nt, synthetic construct
  source 1..20: mol_type = other RNA
tctcaccatttgctttccca

SEQ ID NO: 4734 - RNA, 20 nt, synthetic construct
  source 1..20: mol_type = other RNA
tttgaccctgggaaagcaaa

SEQ ID NO: 4735 - RNA, 20 nt, synthetic construct
  source 1..20: mol_type = other RNA
tgattgtggtttttgaccct

SEQ ID NO: 4736 - RNA, 20 nt, synthetic construct
  source 1..20: mol_type = other RNA
atgattgtggtttttgaccc

SEQ ID NO: 4737 - RNA, 20 nt, synthetic construct
  source 1..20: mol_type = other RNA
cacaatcatcttgataaaca

SEQ ID NO: 4738 - RNA, 20 nt, synthetic construct
  source 1..20: mol_type = other RNA
cttgtttatcaagatgattg

SEQ ID NO: 4739 - RNA, 20 nt, synthetic construct
  source 1..20: mol_type = other RNA
atgtatttttgtatttgcat

SEQ ID NO: 4740 - RNA, 20 nt, synthetic construct
  source 1..20: mol_type = other RNA
aatgggatggaggtgagtgc

SEQ ID NO: 4741 - RNA, 20 nt, synthetic construct
  source 1..20: mol_type = other RNA
gcatattagaaatgggatgg

SEQ ID NO: 4742 - RNA, 20 nt, synthetic construct
  source 1..20: mol_type = other RNA
gttgcatattagaaatggga

SEQ ID NO: 4743 - RNA, 20 nt, synthetic construct
  source 1..20: mol_type = other RNA
atacgttgcatattagaaat

SEQ ID NO: 4744 - RNA, 20 nt, synthetic construct
  source 1..20: mol_type = other RNA
aatacgttgcatattagaaa

SEQ ID NO: 4745 - RNA, 20 nt, synthetic construct
  source 1..20: mol_type = other RNA
agatgcttttcacaatgagt

SEQ ID NO: 4746 - RNA, 20 nt, synthetic construct
  source 1..20: mol_type = other RNA
atacatcagctagccagaaa

SEQ ID NO: 4747 - RNA, 20 nt, synthetic construct
  source 1..20: mol_type = other RNA
tacatcagctagccagaaaa

SEQ ID NO: 4748 - RNA, 20 nt, synthetic construct
  source 1..20: mol_type = other RNA
acatcagctagccagaaaag

SEQ ID NO: 4749 - RNA, 20 nt, synthetic construct
  source 1..20: mol_type = other RNA
tcagctagccagaaaagggg

SEQ ID NO: 4750 - RNA, 20 nt, synthetic construct
  source 1..20: mol_type = other RNA
cattatctcctccccttttc

SEQ ID NO: 4751 - RNA, 20 nt, synthetic construct
  source 1..20: mol_type = other RNA
gagataatgaataataccca

SEQ ID NO: 4752 - RNA, 20 nt, synthetic construct
  source 1..20: mol_type = other RNA
agataatgaataatacccaa

SEQ ID NO: 4753 - RNA, 20 nt, synthetic construct
  source 1..20: mol_type = other RNA
aatgaataatacccaaggga

SEQ ID NO: 4754 - RNA, 20 nt, synthetic construct
  source 1..20: mol_type = other RNA
aaagggattttccttccctt

SEQ ID NO: 4755 - RNA, 20 nt, synthetic construct
  source 1..20: mol_type = other RNA
aaaagggattttccttccct

SEQ ID NO: 4756 - RNA, 20 nt, synthetic construct
  source 1..20: mol_type = other RNA
aggaaaatccctttttcagc

SEQ ID NO: 4757 - RNA, 20 nt, synthetic construct
  source 1..20: mol_type = other RNA
gacttaaaccagctgaaaaa

SEQ ID NO: 4758 - RNA, 20 nt, synthetic construct
  source 1..20: mol_type = other RNA
tgacttaaaccagctgaaaa

SEQ ID NO: 4759 - RNA, 20 nt, synthetic construct
  source 1..20: mol_type = other RNA
tagtgctgtgtgcacattat

SEQ ID NO: 4760 - RNA, 20 nt, synthetic construct
  source 1..20: mol_type = other RNA
gaactaattgaaaagcttta

SEQ ID NO: 4761 - RNA, 20 nt, synthetic construct
  source 1..20: mol_type = other RNA
tatattttctgggagttaga

SEQ ID NO: 4762 - RNA, 20 nt, synthetic construct
  source 1..20: mol_type = other RNA
gtgcgtgaattatattttct

SEQ ID NO: 4763 - RNA, 20 nt, synthetic construct
  source 1..20: mol_type = other RNA
tgtgcgtgaattatattttc

SEQ ID NO: 4764 - RNA, 20 nt, synthetic construct
  source 1..20: mol_type = other RNA
atagctagcaggatgctgtg

SEQ ID NO: 4765 - RNA, 20 nt, synthetic construct
  source 1..20: mol_type = other RNA
aatgatggataatagctagc

SEQ ID NO: 4766 - RNA, 20 nt, synthetic construct
  source 1..20: mol_type = other RNA
caaataacacttgtaaatga

SEQ ID NO: 4767 - RNA, 20 nt, synthetic construct
  source 1..20: mol_type = other RNA
cactaaagttttgaaaaacg

SEQ ID NO: 4768 - RNA, 20 nt, synthetic construct
  source 1..20: mol_type = other RNA
gaggctgctctgccttcttc

SEQ ID NO: 4769 - RNA, 20 nt, synthetic construct
  source 1..20: mol_type = other RNA
gttaaaacacagccagaaga

SEQ ID NO: 4770 - RNA, 20 nt, synthetic construct
  source 1..20: mol_type = other RNA
tctggctgtgttttaacaaa

SEQ ID NO: 4771 - RNA, 20 nt, synthetic construct
  source 1..20: mol_type = other RNA
acaaatggtatcaatgcaaa

SEQ ID NO: 4772 - RNA, 20 nt, synthetic construct
  source 1..20: mol_type = other RNA
gagcaataaatttttttaaa

SEQ ID NO: 4773 - RNA, 20 nt, synthetic construct
  source 1..20: mol_type = other RNA
agacatttggctatctagac

SEQ ID NO: 4774 - RNA, 20 nt, synthetic construct
  source 1..20: mol_type = other RNA
tgtatcagccttcagacatt

SEQ ID NO: 4775 - RNA, 20 nt, synthetic construct
  source 1..20: mol_type = other RNA
ggctgatacacaatgaaata

SEQ ID NO: 4776 - RNA, 20 nt, synthetic construct
  source 1..20: mol_type = other RNA
gctgatacacaatgaaataa

SEQ ID NO: 4777 - RNA, 20 nt, synthetic construct
  source 1..20: mol_type = other RNA
tttagagataatgatcttta

SEQ ID NO: 4778 - RNA, 20 nt, synthetic construct
  source 1..20: mol_type = other RNA
ttttagagataatgatcttt

SEQ ID NO: 4779 - RNA, 20 nt, synthetic construct
  source 1..20: mol_type = other RNA
ttttatgcatctctttttgc

SEQ ID NO: 4780 - RNA, 20 nt, synthetic construct
  source 1..20: mol_type = other RNA
aaacagtttatgttgtaaaa

SEQ ID NO: 4781 - RNA, 20 nt, synthetic construct
  source 1..20: mol_type = other RNA
aaaacagtttatgttgtaaa

SEQ ID NO: 4782 - RNA, 20 nt, synthetic construct
  source 1..20: mol_type = other RNA
ttagtcatggttgtcagttg

SEQ ID NO: 4783 - RNA, 20 nt, synthetic construct
  source 1..20: mol_type = other RNA
atgactaaaacatgaattct

SEQ ID NO: 4784 - RNA, 20 nt, synthetic construct
  source 1..20: mol_type = other RNA
tagaattcatgttttagtca

SEQ ID NO: 4785 - RNA, 20 nt, synthetic construct
  source 1..20: mol_type = other RNA
gattaacattaaaataattt

SEQ ID NO: 4786 - RNA, 20 nt, synthetic construct
  source 1..20: mol_type = other RNA
attaacattaaaataatttt

SEQ ID NO: 4787 - RNA, 20 nt, synthetic construct
  source 1..20: mol_type = other RNA
ttaaaataattttgggacag

SEQ ID NO: 4788 - RNA, 20 nt, synthetic construct
  source 1..20: mol_type = other RNA
taaaataattttgggacaga

SEQ ID NO: 4789 - RNA, 20 nt, synthetic construct
  source 1..20: mol_type = other RNA
cccttccatttttcttttgc

SEQ ID NO: 4790 - RNA, 20 nt, synthetic construct
  source 1..20: mol_type = other RNA
ccagcaaaagaaaaatggaa

SEQ ID NO: 4791 - RNA, 20 nt, synthetic construct
  source 1..20: mol_type = other RNA
accagcaaaagaaaaatgga

SEQ ID NO: 4792 - RNA, 20 nt, synthetic construct
  source 1..20: mol_type = other RNA
agataccagcaaaagaaaaa

SEQ ID NO: 4793 - RNA, 20 nt, synthetic construct
  source 1..20: mol_type = other RNA
aagaacaaaactagtgtagg

SEQ ID NO: 4794 - RNA, 20 nt, synthetic construct
  source 1..20: mol_type = other RNA
tggaagaacaaaactagtgt

SEQ ID NO: 4795 - RNA, 20 nt, synthetic construct
  source 1..20: mol_type = other RNA
tttgagaatagatttttgag

SEQ ID NO: 4796 - RNA, 20 nt, synthetic construct
  source 1..20: mol_type = other RNA
tgcattatcttcaagtagtt

SEQ ID NO: 4797 - RNA, 20 nt, synthetic construct
  source 1..20: mol_type = other RNA
aattttatatcttcttttct

SEQ ID NO: 4798 - RNA, 20 nt, synthetic construct
  source 1..20: mol_type = other RNA
cagctgtctgctggcatgat

SEQ ID NO: 4799 - RNA, 20 nt, synthetic construct
  source 1..20: mol_type = other RNA
taataatgtcagctgtctgc

SEQ ID NO: 4800 - RNA, 20 nt, synthetic construct
  source 1..20: mol_type = other RNA
agcaagaaaagaaatgaaga

SEQ ID NO: 4801 - RNA, 20 nt, synthetic construct
  source 1..20: mol_type = other RNA
tgaagaaggcaattatatag

SEQ ID NO: 4802 - RNA, 20 nt, synthetic construct
  source 1..20: mol_type = other RNA
tgactacaaatgtgcttctt

SEQ ID NO: 4803 - RNA, 20 nt, synthetic construct
  source 1..20: mol_type = other RNA
ttgactacaaatgtgcttct

SEQ ID NO: 4804 - RNA, 20 nt, synthetic construct
  source 1..20: mol_type = other RNA
gctaaacagtagttcactcg

SEQ ID NO: 4805 - RNA, 20 nt, synthetic construct
  source 1..20: mol_type = other RNA
ctccccctgccagatatttt

SEQ ID NO: 4806 - RNA, 20 nt, synthetic construct
  source 1..20: mol_type = other RNA
tccccctgccagatattttt

SEQ ID NO: 4807 - RNA, 20 nt, synthetic construct
  source 1..20: mol_type = other RNA
ccccctgccagatatttttg

SEQ ID NO: 4808 - RNA, 20 nt, synthetic construct
  source 1..20: mol_type = other RNA
aaaaatatctggcaggggga

SEQ ID NO: 4809 - RNA, 20 nt, synthetic construct
  source 1..20: mol_type = other RNA
caaaaatatctggcaggggg

SEQ ID NO: 4810 - RNA, 20 nt, synthetic construct
  source 1..20: mol_type = other RNA
ccccaaaaatatctggcagg

SEQ ID NO: 4811 - RNA, 20 nt, synthetic construct
  source 1..20: mol_type = other RNA
accccaaaaatatctggcag

SEQ ID NO: 4812 - RNA, 20 nt, synthetic construct
  source 1..20: mol_type = other RNA
aaccccaaaaatatctggca

SEQ ID NO: 4813 - RNA, 20 nt, synthetic construct
  source 1..20: mol_type = other RNA
caaccccaaaaatatctggc

SEQ ID NO: 4814 - RNA, 20 nt, synthetic construct
  source 1..20: mol_type = other RNA
ctcacaaccccaaaaatatc

SEQ ID NO: 4815 - RNA, 20 nt, synthetic construct
  source 1..20: mol_type = other RNA
ttttggggttgtgagttttg

SEQ ID NO: 4816 - RNA, 20 nt, synthetic construct
  source 1..20: mol_type = other RNA
tttggggttgtgagttttga

SEQ ID NO: 4817 - RNA, 20 nt, synthetic construct
  source 1..20: mol_type = other RNA
ttggggttgtgagttttgag

SEQ ID NO: 4818 - RNA, 20 nt, synthetic construct
  source 1..20: mol_type = other RNA
acagttcattgatttcttgc

SEQ ID NO: 4819 - RNA, 20 nt, synthetic construct
  source 1..20: mol_type = other RNA
actcattttactgtttactt

SEQ ID NO: 4820 - RNA, 20 nt, synthetic construct
  source 1..20: mol_type = other RNA
ttttatagcttaatgtcata

SEQ ID NO: 4821 - RNA, 20 nt, synthetic construct
  source 1..20: mol_type = other RNA
taaaatagtactgaatcaaa

SEQ ID NO: 4822 - RNA, 20 nt, synthetic construct
  source 1..20: mol_type = other RNA
aaacggagagtagaatactt

SEQ ID NO: 4823 - RNA, 20 nt, synthetic construct
  source 1..20: mol_type = other RNA
cggagagtagaatactttgg

SEQ ID NO: 4824 - RNA, 20 nt, synthetic construct
  source 1..20: mol_type = other RNA
gagtagaatactttggagga

SEQ ID NO: 4825 - RNA, 20 nt, synthetic construct
  source 1..20: mol_type = other RNA
agtagaatactttggaggaa

SEQ ID NO: 4826 - RNA, 20 nt, synthetic construct
  source 1..20: mol_type = other RNA
gtagaatactttggaggaag

SEQ ID NO: 4827 - RNA, 20 nt, synthetic construct
  source 1..20: mol_type = other RNA
gaatactttggaggaagggg

SEQ ID NO: 4828 - RNA, 20 nt, synthetic construct
  source 1..20: mol_type = other RNA
tctgaatatctatagacatt

SEQ ID NO: 4829 - RNA, 20 nt, synthetic construct
  source 1..20: mol_type = other RNA
ccagtgacgaatgaagacac

SEQ ID NO: 4830 - RNA, 20 nt, synthetic construct
  source 1..20: mol_type = other RNA
cagtgacgaatgaagacaca

SEQ ID NO: 4831 - RNA, 20 nt, synthetic construct
  source 1..20: mol_type = other RNA
cctgtgtcttcattcgtcac

SEQ ID NO: 4832 - RNA, 20 nt, synthetic construct
  source 1..20: mol_type = other RNA
acagggaactgagctgagct

SEQ ID NO: 4833 - RNA, 20 nt, synthetic construct
  source 1..20: mol_type = other RNA
gcagggaacagaagagggtg

SEQ ID NO: 4834 - RNA, 20 nt, synthetic construct
  source 1..20: mol_type = other RNA
aagtggcagggaacagaaga

SEQ ID NO: 4835 - RNA, 20 nt, synthetic construct
  source 1..20: mol_type = other RNA
caagtggcagggaacagaag

SEQ ID NO: 4836 - RNA, 20 nt, synthetic construct
  source 1..20: mol_type = other RNA
tggctcttattcaagtggca

SEQ ID NO: 4837 - RNA, 20 nt, synthetic construct
  source 1..20: mol_type = other RNA
ttggctcttattcaagtggc

SEQ ID NO: 4838 - RNA, 20 nt, synthetic construct
  source 1..20: mol_type = other RNA
cattttggctcttattcaag

SEQ ID NO: 4839 - RNA, 20 nt, synthetic construct
  source 1..20: mol_type = other RNA
taagattagaagtggcattt

SEQ ID NO: 4840 - RNA, 20 nt, synthetic construct
  source 1..20: mol_type = other RNA
atggaaaataagattagaag

SEQ ID NO: 4841 - RNA, 20 nt, synthetic construct
  source 1..20: mol_type = other RNA
aataaaacacatttaagaaa

SEQ ID NO: 4842 - RNA, 20 nt, synthetic construct
  source 1..20: mol_type = other RNA
atttagctttgcaataaaag

SEQ ID NO: 4843 - RNA, 20 nt, synthetic construct
  source 1..20: mol_type = other RNA
gcaaagctaaatattctaat

SEQ ID NO: 4844 - RNA, 20 nt, synthetic construct
  source 1..20: mol_type = other RNA
tgtaatgctctgcagcagtg

SEQ ID NO: 4845 - RNA, 20 nt, synthetic construct
  source 1..20: mol_type = other RNA
gctctgcagcagtgaggttc

SEQ ID NO: 4846 - RNA, 20 nt, synthetic construct
  source 1..20: mol_type = other RNA
aggttctggcagacccagtg

SEQ ID NO: 4847 - RNA, 20 nt, synthetic construct
  source 1..20: mol_type = other RNA
gaaataaatgggacctcact

SEQ ID NO: 4848 - RNA, 20 nt, synthetic construct
  source 1..20: mol_type = other RNA
agaaataaatgggacctcac

SEQ ID NO: 4849 - RNA, 20 nt, synthetic construct
  source 1..20: mol_type = other RNA
ttacaagtgaagaaataaat

SEQ ID NO: 4850 - RNA, 20 nt, synthetic construct
  source 1..20: mol_type = other RNA
tatttcttcacttgtaataa

SEQ ID NO: 4851 - RNA, 20 nt, synthetic construct
  source 1..20: mol_type = other RNA
tgtgttctgatgcactactc

SEQ ID NO: 4852 - RNA, 20 nt, synthetic construct
  source 1..20: mol_type = other RNA
tcaaagcaatataactaaga

SEQ ID NO: 4853 - RNA, 20 nt, synthetic construct
  source 1..20: mol_type = other RNA
atcctttctactcattcaaa

SEQ ID NO: 4854 - RNA, 20 nt, synthetic construct
  source 1..20: mol_type = other RNA
ctccttttgaatgagtagaa

SEQ ID NO: 4855 - RNA, 20 nt, synthetic construct
  source 1..20: mol_type = other RNA
acaatgctgattattcctga

SEQ ID NO: 4856 - RNA, 20 nt, synthetic construct
  source 1..20: mol_type = other RNA
caggaataatcagcattgtt

SEQ ID NO: 4857 - RNA, 20 nt, synthetic construct
  source 1..20: mol_type = other RNA
tgaaaatcaaaaggtccttc

SEQ ID NO: 4858 - RNA, 20 nt, synthetic construct
  source 1..20: mol_type = other RNA
caaatgctttgaaaatcaaa

SEQ ID NO: 4859 - RNA, 20 nt, synthetic construct
  source 1..20: mol_type = other RNA
atccacgcagcccctccgca

SEQ ID NO: 4860 - RNA, 20 nt, synthetic construct
  source 1..20: mol_type = other RNA
ttccttgcggaggggctgcg

SEQ ID NO: 4861 - RNA, 20 nt, synthetic construct
  source 1..20: mol_type = other RNA
ccctccgcaaggaaaactag

SEQ ID NO: 4862 - RNA, 20 nt, synthetic construct
  source 1..20: mol_type = other RNA
ctctagttttccttgcggag

SEQ ID NO: 4863 - RNA, 20 nt, synthetic construct
  source 1..20: mol_type = other RNA
cctctagttttccttgcgga

SEQ ID NO: 4864 - RNA, 20 nt, synthetic construct
  source 1..20: mol_type = other RNA
tcctctagttttccttgcgg

SEQ ID NO: 4865 - RNA, 20 nt, synthetic construct
  source 1..20: mol_type = other RNA
ttctcctctagttttccttg

SEQ ID NO: 4866 - RNA, 20 nt, synthetic construct
  source 1..20: mol_type = other RNA
aacattttagagacaacaac

SEQ ID NO: 4867 - RNA, 20 nt, synthetic construct
  source 1..20: mol_type = other RNA
attttagagacaacaacagg

SEQ ID NO: 4868 - RNA, 20 nt, synthetic construct
  source 1..20: mol_type = other RNA
ttttagagacaacaacagga

SEQ ID NO: 4869 - RNA, 20 nt, synthetic construct
  source 1..20: mol_type = other RNA
tttagagacaacaacaggag

SEQ ID NO: 4870 - RNA, 20 nt, synthetic construct
  source 1..20: mol_type = other RNA
aacaggaggggacagatatt

SEQ ID NO: 4871 - RNA, 20 nt, synthetic construct
  source 1..20: mol_type = other RNA
gaagctctcagacttttgtc

SEQ ID NO: 4872 - RNA, 20 nt, synthetic construct
  source 1..20: mol_type = other RNA
aatcaagtgacattttctgc

SEQ ID NO: 4873 - RNA, 20 nt, synthetic construct
  source 1..20: mol_type = other RNA
tgattcatatcttcaactcc

SEQ ID NO: 4874 - RNA, 20 nt, synthetic construct
  source 1..20: mol_type = other RNA
gattcatatcttcaactcca

SEQ ID NO: 4875 - RNA, 20 nt, synthetic construct
  source 1..20: mol_type = other RNA
actccagggttatgccctga

SEQ ID NO: 4876 - RNA, 20 nt, synthetic construct
  source 1..20: mol_type = other RNA
tttccttcagggcataaccc

SEQ ID NO: 4877 - RNA, 20 nt, synthetic construct
  source 1..20: mol_type = other RNA
tcatgagtgcatttccttca

SEQ ID NO: 4878 - RNA, 20 nt, synthetic construct
  source 1..20: mol_type = other RNA
atcatgagtgcatttccttc

SEQ ID NO: 4879 - RNA, 20 nt, synthetic construct
  source 1..20: mol_type = other RNA
atgatgtgaactgcaattcg

SEQ ID NO: 4880 - RNA, 20 nt, synthetic construct
  source 1..20: mol_type = other RNA
ggaatgaattatgggtaaga

SEQ ID NO: 4881 - RNA, 20 nt, synthetic construct
  source 1..20: mol_type = other RNA
ggtaagggggaatgaattat

SEQ ID NO: 4882 - RNA, 20 nt, synthetic construct
  source 1..20: mol_type = other RNA
aggtaagggggaatgaatta

SEQ ID NO: 4883 - RNA, 20 nt, synthetic construct
  source 1..20: mol_type = other RNA
ttaaagtgtgctaggtaagg

SEQ ID NO: 4884 - RNA, 20 nt, synthetic construct
  source 1..20: mol_type = other RNA
cttaaagtgtgctaggtaag

SEQ ID NO: 4885 - RNA, 20 nt, synthetic construct
  source 1..20: mol_type = other RNA
tcttaaagtgtgctaggtaa

SEQ ID NO: 4886 - RNA, 20 nt, synthetic construct
  source 1..20: mol_type = other RNA
atcttaaagtgtgctaggta

SEQ ID NO: 4887 - RNA, 20 nt, synthetic construct
  source 1..20: mol_type = other RNA
aacagatcttaaagtgtgct

SEQ ID NO: 4888 - RNA, 20 nt, synthetic construct
  source 1..20: mol_type = other RNA
tttttttttttttaactatg

SEQ ID NO: 4889 - RNA, 20 nt, synthetic construct
  source 1..20: mol_type = other RNA
agttaaaaaaaaaaaaaaaa

SEQ ID NO: 4890 - RNA, 20 nt, synthetic construct
  source 1..20: mol_type = other RNA
taaaaaaaaaaaaaaaaagg

SEQ ID NO: 4891 - RNA, 20 nt, synthetic construct
  source 1..20: mol_type = other RNA
aaaaaaaaaaaaaaaaaggt

SEQ ID NO: 4892 - RNA, 20 nt, synthetic construct
  source 1..20: mol_type = other RNA
aaaaaaaaaaaaaaaaggtg

SEQ ID NO: 4893 - RNA, 20 nt, synthetic construct
  source 1..20: mol_type = other RNA
aaaaaaaaaaaaaaaggtgg

SEQ ID NO: 4894 - RNA, 20 nt, synthetic construct
  source 1..20: mol_type = other RNA
aaaaaaaaaaaaaaggtggg

SEQ ID NO: 4895 - RNA, 20 nt, synthetic construct
  source 1..20: mol_type = other RNA
aaaaaaaaaaaggtgggggg

SEQ ID NO: 4896 - RNA, 20 nt, synthetic construct
  source 1..20: mol_type = other RNA
aaaaaaaaaaggtgggggga

SEQ ID NO: 4897 - RNA, 20 nt, synthetic construct
  source 1..20: mol_type = other RNA
tcctaaacccctttcgtccc

SEQ ID NO: 4898 - RNA, 20 nt, synthetic construct
  source 1..20: mol_type = other RNA
tcctgggacgaaaggggttt

SEQ ID NO: 4899 - RNA, 20 nt, synthetic construct
  source 1..20: mol_type = other RNA
tctaagtcctgggacgaaag

SEQ ID NO: 4900 - RNA, 20 nt, synthetic construct
  source 1..20: mol_type = other RNA
ttctaagtcctgggacgaaa

SEQ ID NO: 4901 - RNA, 20 nt, synthetic construct
  source 1..20: mol_type = other RNA
tttctaagtcctgggacgaa

SEQ ID NO: 4902 - RNA, 20 nt, synthetic construct
  source 1..20: mol_type = other RNA
aaataagctttctaagtcct

SEQ ID NO: 4903 - RNA, 20 nt, synthetic construct
  source 1..20: mol_type = other RNA
aaaataagctttctaagtcc

SEQ ID NO: 4904 - RNA, 20 nt, synthetic construct
  source 1..20: mol_type = other RNA
ccagtccaatatacagccaa

SEQ ID NO: 4905 - RNA, 20 nt, synthetic construct
  source 1..20: mol_type = other RNA
tccaatatacagccaaagga

SEQ ID NO: 4906 - RNA, 20 nt, synthetic construct
  source 1..20: mol_type = other RNA
cctttggctgtatattggac

SEQ ID NO: 4907 - RNA, 20 nt, synthetic construct
  source 1..20: mol_type = other RNA
atacagccaaaggaaggagc

SEQ ID NO: 4908 - RNA, 20 nt, synthetic construct
  source 1..20: mol_type = other RNA
gattatcctgctccttcctt

SEQ ID NO: 4909 - RNA, 20 nt, synthetic construct
  source 1..20: mol_type = other RNA
aaggagcaggataatctaca

SEQ ID NO: 4910 - RNA, 20 nt, synthetic construct
  source 1..20: mol_type = other RNA
aggagcaggataatctacaa

SEQ ID NO: 4911 - RNA, 20 nt, synthetic construct
  source 1..20: mol_type = other RNA
tcaggaaggaaacagataag

SEQ ID NO: 4912 - RNA, 20 nt, synthetic construct
  source 1..20: mol_type = other RNA
gtttccttcctgagaacaaa

SEQ ID NO: 4913 - RNA, 20 nt, synthetic construct
  source 1..20: mol_type = other RNA
tggtccatttgttctcagga

SEQ ID NO: 4914 - RNA, 20 nt, synthetic construct
  source 1..20: mol_type = other RNA
tgcttggtccatttgttctc

SEQ ID NO: 4915 - RNA, 20 nt, synthetic construct
  source 1..20: mol_type = other RNA
tacactcacatctgtatgct

SEQ ID NO: 4916 - RNA, 20 nt, synthetic construct
  source 1..20: mol_type = other RNA
cttcagatgcactttgagag

SEQ ID NO: 4917 - RNA, 20 nt, synthetic construct
  source 1..20: mol_type = other RNA
acttcagatgcactttgaga

SEQ ID NO: 4918 - RNA, 20 nt, synthetic construct
  source 1..20: mol_type = other RNA
tacttcagatgcactttgag

SEQ ID NO: 4919 - RNA, 20 nt, synthetic construct
  source 1..20: mol_type = other RNA
aacagactgatcactcagaa

SEQ ID NO: 4920 - RNA, 20 nt, synthetic construct
  source 1..20: mol_type = other RNA
tgatcagtctgttccctgaa

SEQ ID NO: 4921 - RNA, 20 nt, synthetic construct
  source 1..20: mol_type = other RNA
cctgaaaggtcagaattttc

SEQ ID NO: 4922 - RNA, 20 nt, synthetic construct
  source 1..20: mol_type = other RNA
cagaaaattctgacctttca

SEQ ID NO: 4923 - RNA, 20 nt, synthetic construct
  source 1..20: mol_type = other RNA
ccagaaaattctgacctttc

SEQ ID NO: 4924 - RNA, 20 nt, synthetic construct
  source 1..20: mol_type = other RNA
ttgttgctgtttagacaggg

SEQ ID NO: 4925 - RNA, 20 nt, synthetic construct
  source 1..20: mol_type = other RNA
tcgttgttgctgtttagaca

SEQ ID NO: 4926 - RNA, 20 nt, synthetic construct
  source 1..20: mol_type = other RNA
gtcgttgttgctgtttagac

SEQ ID NO: 4927 - RNA, 20 nt, synthetic construct
  source 1..20: mol_type = other RNA
ttccattgataagccaatag

SEQ ID NO: 4928 - RNA, 20 nt, synthetic construct
  source 1..20: mol_type = other RNA
tgccactattggcttatcaa

SEQ ID NO: 4929 - RNA, 20 nt, synthetic construct
  source 1..20: mol_type = other RNA
aatagtggcattaataataa

SEQ ID NO: 4930 - RNA, 20 nt, synthetic construct
  source 1..20: mol_type = other RNA
attattattaatgccactat

SEQ ID NO: 4931 - RNA, 20 nt, synthetic construct
  source 1..20: mol_type = other RNA
tctagatatcttaagactct

SEQ ID NO: 4932 - RNA, 20 nt, synthetic construct
  source 1..20: mol_type = other RNA
gagagggatgataaaaatat

SEQ ID NO: 4933 - RNA, 20 nt, synthetic construct
  source 1..20: mol_type = other RNA
ggagagggatgataaaaata

SEQ ID NO: 4934 - RNA, 20 nt, synthetic construct
  source 1..20: mol_type = other RNA
ttttatcatccctctccatg

SEQ ID NO: 4935 - RNA, 20 nt, synthetic construct
  source 1..20: mol_type = other RNA
atcatccctctccatgaggt

SEQ ID NO: 4936 - RNA, 20 nt, synthetic construct
  source 1..20: mol_type = other RNA
tcatccctctccatgaggta

SEQ ID NO: 4937 - RNA, 20 nt, synthetic construct
  source 1..20: mol_type = other RNA
cctctccatgaggtagggca

SEQ ID NO: 4938 - RNA, 20 nt, synthetic construct
  source 1..20: mol_type = other RNA
ctctccatgaggtagggcaa

SEQ ID NO: 4939 - RNA, 20 nt, synthetic construct
  source 1..20: mol_type = other RNA
cttgccctacctcatggaga

SEQ ID NO: 4940 - RNA, 20 nt, synthetic construct
  source 1..20: mol_type = other RNA
ccttgccctacctcatggag

SEQ ID NO: 4941 - RNA, 20 nt, synthetic construct
  source 1..20: mol_type = other RNA
agtacccttgccctacctca

SEQ ID NO: 4942 - RNA, 20 nt, synthetic construct
  source 1..20: mol_type = other RNA
catagttctcttgtgaaata

SEQ ID NO: 4943 - RNA, 20 nt, synthetic construct
  source 1..20: mol_type = other RNA
acatagttctcttgtgaaat

SEQ ID NO: 4944 - RNA, 20 nt, synthetic construct
  source 1..20: mol_type = other RNA
gacaagtcttttaattttct

SEQ ID NO: 4945 - RNA, 20 nt, synthetic construct
  source 1..20: mol_type = other RNA
gacttgtctaagctctaaac

SEQ ID NO: 4946 - RNA, 20 nt, synthetic construct
  source 1..20: mol_type = other RNA
taagctctaaactggtaaca

SEQ ID NO: 4947 - RNA, 20 nt, synthetic construct
  source 1..20: mol_type = other RNA
acaaggcagagacatgaatt

SEQ ID NO: 4948 - RNA, 20 nt, synthetic construct
  source 1..20: mol_type = other RNA
caaggcagagacatgaattt

SEQ ID NO: 4949 - RNA, 20 nt, synthetic construct
  source 1..20: mol_type = other RNA
actctctgctaactaaataa

SEQ ID NO: 4950 - RNA, 20 nt, synthetic construct
  source 1..20: mol_type = other RNA
tatttagttagcagagagtt

SEQ ID NO: 4951 - RNA, 20 nt, synthetic construct
  source 1..20: mol_type = other RNA
ttgacttttgtatgtcttct

SEQ ID NO: 4952 - RNA, 20 nt, synthetic construct
  source 1..20: mol_type = other RNA
gttgacttttgtatgtcttc

SEQ ID NO: 4953 - RNA, 20 nt, synthetic construct
  source 1..20: mol_type = other RNA
taggcagtgtaaataacagc

SEQ ID NO: 4954 - RNA, 20 nt, synthetic construct
  source 1..20: mol_type = other RNA
ctggaacaaacatttattgt

SEQ ID NO: 4955 - RNA, 20 nt, synthetic construct
  source 1..20: mol_type = other RNA
cttgtttgaactattttttc

SEQ ID NO: 4956 - RNA, 20 nt, synthetic construct
  source 1..20: mol_type = other RNA
agaaatagtttaaacacaaa

SEQ ID NO: 4957 - RNA, 20 nt, synthetic construct
  source 1..20: mol_type = other RNA
gtttaaacacaaaaggctga

SEQ ID NO: 4958 - RNA, 20 nt, synthetic construct
  source 1..20: mol_type = other RNA
tttaaacacaaaaggctgaa

SEQ ID NO: 4959 - RNA, 20 nt, synthetic construct
  source 1..20: mol_type = other RNA
aaggctgaagggttcaatat

SEQ ID NO: 4960 - RNA, 20 nt, synthetic construct
  source 1..20: mol_type = other RNA
tatgtttgcttttaatacag

SEQ ID NO: 4961 - RNA, 20 nt, synthetic construct
  source 1..20: mol_type = other RNA
gtttgcttttaatacagtgg

SEQ ID NO: 4962 - RNA, 20 nt, synthetic construct
  source 1..20: mol_type = other RNA
atacagtggaggaactgttc

SEQ ID NO: 4963 - RNA, 20 nt, synthetic construct
  source 1..20: mol_type = other RNA
aacagtttgttcttctgtaa

SEQ ID NO: 4964 - RNA, 20 nt, synthetic construct
  source 1..20: mol_type = other RNA
gtttgttcttctgtaaaggc

SEQ ID NO: 4965 - RNA, 20 nt, synthetic construct
  source 1..20: mol_type = other RNA
tggccttgttgtactgccga

SEQ ID NO: 4966 - RNA, 20 nt, synthetic construct
  source 1..20: mol_type = other RNA
cggccttcggcagtacaaca

SEQ ID NO: 4967 - RNA, 20 nt, synthetic construct
  source 1..20: mol_type = other RNA
gcttgtgatcttgcggcctt

SEQ ID NO: 4968 - RNA, 20 nt, synthetic construct
  source 1..20: mol_type = other RNA
ccgcaagatcacaagctacg

SEQ ID NO: 4969 - RNA, 20 nt, synthetic construct
  source 1..20: mol_type = other RNA
ccacgtagcttgtgatcttg

SEQ ID NO: 4970 - RNA, 20 nt, synthetic construct
  source 1..20: mol_type = other RNA
attgagacgccagctcgctt

SEQ ID NO: 4971 - RNA, 20 nt, synthetic construct
  source 1..20: mol_type = other RNA
ttggttgtgccgaagcgagc

SEQ ID NO: 4972 - RNA, 20 nt, synthetic construct
  source 1..20: mol_type = other RNA
tagagcattaagagagaagt

SEQ ID NO: 4973 - RNA, 20 nt, synthetic construct
  source 1..20: mol_type = other RNA
gtcaaagctatgaagaagac

SEQ ID NO: 4974 - RNA, 20 nt, synthetic construct
  source 1..20: mol_type = other RNA
aaaaagatcattcatggttc

SEQ ID NO: 4975 - RNA, 20 nt, synthetic construct
  source 1..20: mol_type = other RNA
tttgtcaaaaagatcattca

SEQ ID NO: 4976 - RNA, 20 nt, synthetic construct
  source 1..20: mol_type = other RNA
tttaaatgtgtgttataaac

SEQ ID NO: 4977 - RNA, 20 nt, synthetic construct
  source 1..20: mol_type = other RNA
ttaaatgtgtgttataaaca

SEQ ID NO: 4978 - RNA, 20 nt, synthetic construct
  source 1..20: mol_type = other RNA
aagtgtcctaattttgatac

SEQ ID NO: 4979 - RNA, 20 nt, synthetic construct
  source 1..20: mol_type = other RNA
agtgtcctaattttgataca

SEQ ID NO: 4980 - RNA, 20 nt, synthetic construct
  source 1..20: mol_type = other RNA
tagcaccctgtatcaaaatt

SEQ ID NO: 4981 - RNA, 20 nt, synthetic construct
  source 1..20: mol_type = other RNA
ctaagaaatacagaaaacaa

SEQ ID NO: 4982 - RNA, 20 nt, synthetic construct
  source 1..20: mol_type = other RNA
agaaaacaaaggaaattaac

SEQ ID NO: 4983 - RNA, 20 nt, synthetic construct
  source 1..20: mol_type = other RNA
gaaaacaaaggaaattaact

SEQ ID NO: 4984 - RNA, 20 nt, synthetic construct
  source 1..20: mol_type = other RNA
ggaaattaactgggagatcc

SEQ ID NO: 4985 - RNA, 20 nt, synthetic construct
  source 1..20: mol_type = other RNA
gaaattaactgggagatcca

SEQ ID NO: 4986 - RNA, 20 nt, synthetic construct
  source 1..20: mol_type = other RNA
attaactgggagatccaggg

SEQ ID NO: 4987 - RNA, 20 nt, synthetic construct
  source 1..20: mol_type = other RNA
agattgtttcttagcctccc

SEQ ID NO: 4988 - RNA, 20 nt, synthetic construct
  source 1..20: mol_type = other RNA
gctaagaaacaatctgccac

SEQ ID NO: 4989 - RNA, 20 nt, synthetic construct
  source 1..20: mol_type = other RNA
ctaagaaacaatctgccact

SEQ ID NO: 4990 - RNA, 20 nt, synthetic construct
  source 1..20: mol_type = other RNA
gctatggctgtttctcccag

SEQ ID NO: 4991 - RNA, 20 nt, synthetic construct
  source 1..20: mol_type = other RNA
gccatagcttctgatgagct

SEQ ID NO: 4992 - RNA, 20 nt, synthetic construct
  source 1..20: mol_type = other RNA
tcctagctcatcagaagcta

SEQ ID NO: 4993 - RNA, 20 nt, synthetic construct
  source 1..20: mol_type = other RNA
gatgagctaggaagattttg

SEQ ID NO: 4994 - RNA, 20 nt, synthetic construct
  source 1..20: mol_type = other RNA
gatatcacagctgtttgttg

SEQ ID NO: 4995 - RNA, 20 nt, synthetic construct
  source 1..20: mol_type = other RNA
acagctgtttgttgaggctg

SEQ ID NO: 4996 - RNA, 20 nt, synthetic construct
  source 1..20: mol_type = other RNA
gctgtttgttgaggctgtgg

SEQ ID NO: 4997 - RNA, 20 nt, synthetic construct
  source 1..20: mol_type = other RNA
ctgtttgttgaggctgtggt

SEQ ID NO: 4998 - RNA, 20 nt, synthetic construct
  source 1..20: mol_type = other RNA
ggtgggatttctttttcaag

SEQ ID NO: 4999 - RNA, 20 nt, synthetic construct
  source 1..20: mol_type = other RNA
gtgggatttctttttcaaga

SEQ ID NO: 5000 - RNA, 20 nt, synthetic construct
  source 1..20: mol_type = other RNA
tttctttttcaagagggtga

SEQ ID NO: 5001 - RNA, 20 nt, synthetic construct
  source 1..20: mol_type = other RNA
ttctttttcaagagggtgaa

SEQ ID NO: 5002 - RNA, 20 nt, synthetic construct
  source 1..20: mol_type = other RNA
ggtgaagggagatttgaact

SEQ ID NO: 5003 - RNA, 20 nt, synthetic construct
  source 1..20: mol_type = other RNA
tgacacaattatcctaaagt

SEQ ID NO: 5004 - RNA, 20 nt, synthetic construct
  source 1..20: mol_type = other RNA
tactttaggataattgtgtc

SEQ ID NO: 5005 - RNA, 20 nt, synthetic construct
  source 1..20: mol_type = other RNA
taaagtaggaaagcctcagt

SEQ ID NO: 5006 - RNA, 20 nt, synthetic construct
  source 1..20: mol_type = other RNA
aactgaggctttcctacttt

SEQ ID NO: 5007 - RNA, 20 nt, synthetic construct
  source 1..20: mol_type = other RNA
aggaaagcctcagttggaag

SEQ ID NO: 5008 - RNA, 20 nt, synthetic construct
  source 1..20: mol_type = other RNA
aactcatcctcttccaactg

SEQ ID NO: 5009 - RNA, 20 nt, synthetic construct
  source 1..20: mol_type = other RNA
agtttctttaaatagcccaa

SEQ ID NO: 5010 - RNA, 20 nt, synthetic construct
  source 1..20: mol_type = other RNA
aaggctgtgatgcgtaaaaa

SEQ ID NO: 5011 - RNA, 20 nt, synthetic construct
  source 1..20: mol_type = other RNA
ttttacgcatcacagccttt

SEQ ID NO: 5012 - RNA, 20 nt, synthetic construct
  source 1..20: mol_type = other RNA
tttttacgcatcacagcctt

SEQ ID NO: 5013 - RNA, 20 nt, synthetic construct
  source 1..20: mol_type = other RNA
aaaaaggacttgacttattc

SEQ ID NO: 5014 - RNA, 20 nt, synthetic construct
  source 1..20: mol_type = other RNA
cttattctggatagctccag

SEQ ID NO: 5015 - RNA, 20 nt, synthetic construct
  source 1..20: mol_type = other RNA
ttattctggatagctccaga

SEQ ID NO: 5016 - RNA, 20 nt, synthetic construct
  source 1..20: mol_type = other RNA
cagagggcaaaactagcaag

SEQ ID NO: 5017 - RNA, 20 nt, synthetic construct
  source 1..20: mol_type = other RNA
cacttgctagttttgccctc

SEQ ID NO: 5018 - RNA, 20 nt, synthetic construct
  source 1..20: mol_type = other RNA
aaaactagcaagtggccagc

SEQ ID NO: 5019 - RNA, 20 nt, synthetic construct
  source 1..20: mol_type = other RNA
ctgagtatgtgtgttcctgc

SEQ ID NO: 5020 - RNA, 20 nt, synthetic construct
  source 1..20: mol_type = other RNA
agcagagcttgctaataatt

SEQ ID NO: 5021 - RNA, 20 nt, synthetic construct
  source 1..20: mol_type = other RNA
ggactgcctcatccatagca

SEQ ID NO: 5022 - RNA, 20 nt, synthetic construct
  source 1..20: mol_type = other RNA
agtgttccttgctatggatg

SEQ ID NO: 5023 - RNA, 20 nt, synthetic construct
  source 1..20: mol_type = other RNA
ccatagcaaggaacactcag

SEQ ID NO: 5024 - RNA, 20 nt, synthetic construct
  source 1..20: mol_type = other RNA
cctctgagtgttccttgcta

SEQ ID NO: 5025 - RNA, 20 nt, synthetic construct
  source 1..20: mol_type = other RNA
cgtgggggtggggtgggtcg

SEQ ID NO: 5026 - RNA, 20 nt, synthetic construct
  source 1..20: mol_type = other RNA
ccgtgggggtggggtgggtc

SEQ ID NO: 5027 - RNA, 20 nt, synthetic construct
  source 1..20: mol_type = other RNA
gccgtgggggtggggtgggt

SEQ ID NO: 5028 - RNA, 20 nt, synthetic construct
  source 1..20: mol_type = other RNA
caccccacccccacggcggc

SEQ ID NO: 5029 - RNA, 20 nt, synthetic construct
  source 1..20: mol_type = other RNA
ggccgccgtgggggtggggt

SEQ ID NO: 5030 - RNA, 20 nt, synthetic construct
  source 1..20: mol_type = other RNA
cggccgccgtgggggtgggg

SEQ ID NO: 5031 - RNA, 20 nt, synthetic construct
  source 1..20: mol_type = other RNA
ggccggccgccgtgggggtg

SEQ ID NO: 5032 - RNA, 20 nt, synthetic construct
  source 1..20: mol_type = other RNA
ccccacggcggccggccgcc

SEQ ID NO: 5033 - RNA, 20 nt, synthetic construct
  source 1..20: mol_type = other RNA
gcggccggccgccgtggggg

SEQ ID NO: 5034 - RNA, 20 nt, synthetic construct
  source 1..20: mol_type = other RNA
cgggcggccggccgccgtgg

SEQ ID NO: 5035 - RNA, 20 nt, synthetic construct
  source 1..20: mol_type = other RNA
ccgggcggccggccgccgtg

SEQ ID NO: 5036 - RNA, 20 nt, synthetic construct
  source 1..20: mol_type = other RNA
tccgggcggccggccgccgt

SEQ ID NO: 5037 - RNA, 20 nt, synthetic construct
  source 1..20: mol_type = other RNA
ctccgggcggccggccgccg

SEQ ID NO: 5038 - RNA, 20 nt, synthetic construct
  source 1..20: mol_type = other RNA
ggccggccgcccggagcccc

SEQ ID NO: 5039 - RNA, 20 nt, synthetic construct
  source 1..20: mol_type = other RNA
ccgcccggagcccccggccc

SEQ ID NO: 5040 - RNA, 20 nt, synthetic construct
  source 1..20: mol_type = other RNA
ggccgggggctccgggcggc

SEQ ID NO: 5041 - RNA, 20 nt, synthetic construct
  source 1..20: mol_type = other RNA
cctgggccgggggctccggg

SEQ ID NO: 5042 - RNA, 20 nt, synthetic construct
  source 1..20: mol_type = other RNA
tcacctgggccgggggctcc

SEQ ID NO: 5043 - RNA, 20 nt, synthetic construct
  source 1..20: mol_type = other RNA
ctcacctgggccgggggctc

SEQ ID NO: 5044 - RNA, 20 nt, synthetic construct
  source 1..20: mol_type = other RNA
ccggcccaggtgaggacgcg

SEQ ID NO: 5045 - RNA, 20 nt, synthetic construct
  source 1..20: mol_type = other RNA
cggcccaggtgaggacgcgc

SEQ ID NO: 5046 - RNA, 20 nt, synthetic construct
  source 1..20: mol_type = other RNA
cgcgtcctcacctgggccgg

SEQ ID NO: 5047 - RNA, 20 nt, synthetic construct
  source 1..20: mol_type = other RNA
gcgcgtcctcacctgggccg

SEQ ID NO: 5048 - RNA, 20 nt, synthetic construct
  source 1..20: mol_type = other RNA
cgcgcgtcctcacctgggcc

SEQ ID NO: 5049 - RNA, 20 nt, synthetic construct
  source 1..20: mol_type = other RNA
ccgcgcgtcctcacctgggc

SEQ ID NO: 5050 - RNA, 20 nt, synthetic construct
  source 1..20: mol_type = other RNA
cggcccgcgcgtcctcacct

SEQ ID NO: 5051 - RNA, 20 nt, synthetic construct
  source 1..20: mol_type = other RNA
tgaggacgcgcgggccgccg

SEQ ID NO: 5052 - RNA, 20 nt, synthetic construct
  source 1..20: mol_type = other RNA
gcggcgaggggcggccgcgg

SEQ ID NO: 5053 - RNA, 20 nt, synthetic construct
  source 1..20: mol_type = other RNA
ggagcggcgaggggcggccg

SEQ ID NO: 5054 - RNA, 20 nt, synthetic construct
  source 1..20: mol_type = other RNA
cgggcgggagcggcgagggg

SEQ ID NO: 5055 - RNA, 20 nt, synthetic construct
  source 1..20: mol_type = other RNA
gggcgggcgggagcggcgag

SEQ ID NO: 5056 - RNA, 20 nt, synthetic construct
  source 1..20: mol_type = other RNA
cgggcgggcgggagcggcga

SEQ ID NO: 5057 - RNA, 20 nt, synthetic construct
  source 1..20: mol_type = other RNA
ccgctcccgcccgcccgaag

SEQ ID NO: 5058 - RNA, 20 nt, synthetic construct
  source 1..20: mol_type = other RNA
tcccgcccgcccgaagcggc

SEQ ID NO: 5059 - RNA, 20 nt, synthetic construct
  source 1..20: mol_type = other RNA
ccgcttcgggcgggcgggag

SEQ ID NO: 5060 - RNA, 20 nt, synthetic construct
  source 1..20: mol_type = other RNA
cccgcccgaagcggccggca

SEQ ID NO: 5061 - RNA, 20 nt, synthetic construct
  source 1..20: mol_type = other RNA
ccgcccgaagcggccggcac

SEQ ID NO: 5062 - RNA, 20 nt, synthetic construct
  source 1..20: mol_type = other RNA
cgcccgaagcggccggcacg

SEQ ID NO: 5063 - RNA, 20 nt, synthetic construct
  source 1..20: mol_type = other RNA
ccgtgccggccgcttcgggc

SEQ ID NO: 5064 - RNA, 20 nt, synthetic construct
  source 1..20: mol_type = other RNA
cccgtgccggccgcttcggg

SEQ ID NO: 5065 - RNA, 20 nt, synthetic construct
  source 1..20: mol_type = other RNA
gtccccgtgccggccgcttc

SEQ ID NO: 5066 - RNA, 20 nt, synthetic construct
  source 1..20: mol_type = other RNA
agtccccgtgccggccgctt

SEQ ID NO: 5067 - RNA, 20 nt, synthetic construct
  source 1..20: mol_type = other RNA
actgtggtaagtccccgtgc

SEQ ID NO: 5068 - RNA, 20 nt, synthetic construct
  source 1..20: mol_type = other RNA
ggacttaccacagtgactcg

SEQ ID NO: 5069 - RNA, 20 nt, synthetic construct
  source 1..20: mol_type = other RNA
gtgactcgaggtcccattcc

SEQ ID NO: 5070 - RNA, 20 nt, synthetic construct
  source 1..20: mol_type = other RNA
cgaggtcccattcctggagc

SEQ ID NO: 5071 - RNA, 20 nt, synthetic construct
  source 1..20: mol_type = other RNA
gaggtcccattcctggagca

SEQ ID NO: 5072 - RNA, 20 nt, synthetic construct
  source 1..20: mol_type = other RNA
cttagccctgctccaggaat

SEQ ID NO: 5073 - RNA, 20 nt, synthetic construct
  source 1..20: mol_type = other RNA
acttagccctgctccaggaa

SEQ ID NO: 5074 - RNA, 20 nt, synthetic construct
  source 1..20: mol_type = other RNA
cttcgacttagccctgctcc

SEQ ID NO: 5075 - RNA, 20 nt, synthetic construct
  source 1..20: mol_type = other RNA
ggctaagtcgaagctgtcca

SEQ ID NO: 5076 - RNA, 20 nt, synthetic construct
  source 1..20: mol_type = other RNA
taagtcgaagctgtccatgg

SEQ ID NO: 5077 - RNA, 20 nt, synthetic construct
  source 1..20: mol_type = other RNA
aagtcgaagctgtccatggt

SEQ ID NO: 5078 - RNA, 20 nt, synthetic construct
  source 1..20: mol_type = other RNA
tcgaagctgtccatggtggg

SEQ ID NO: 5079 - RNA, 20 nt, synthetic construct
  source 1..20: mol_type = other RNA
gacgctgacacctcccacca

SEQ ID NO: 5080 - RNA, 20 nt, synthetic construct
  source 1..20: mol_type = other RNA
cgccgctaccgccgccgccg

SEQ ID NO: 5081 - RNA, 20 nt, synthetic construct
  source 1..20: mol_type = other RNA
ggcggcggcggtagcggcgg

SEQ ID NO: 5082 - RNA, 20 nt, synthetic construct
  source 1..20: mol_type = other RNA
ctcggcggcggcggtagcgg

SEQ ID NO: 5083 - RNA, 20 nt, synthetic construct
  source 1..20: mol_type = other RNA
ctaccgccgccgccgaggct

SEQ ID NO: 5084 - RNA, 20 nt, synthetic construct
  source 1..20: mol_type = other RNA
taccgccgccgccgaggctc

SEQ ID NO: 5085 - RNA, 20 nt, synthetic construct
  source 1..20: mol_type = other RNA
agcctcggcggcggcggtag

SEQ ID NO: 5086 - RNA, 20 nt, synthetic construct
  source 1..20: mol_type = other RNA
ggcccgagcctcggcggcgg

SEQ ID NO: 5087 - RNA, 20 nt, synthetic construct
  source 1..20: mol_type = other RNA
ggcggcccgagcctcggcgg

SEQ ID NO: 5088 - RNA, 20 nt, synthetic construct
  source 1..20: mol_type = other RNA
gcgggcggcccgagcctcgg

SEQ ID NO: 5089 - RNA, 20 nt, synthetic construct
  source 1..20: mol_type = other RNA
cgcgcgggcggcccgagcct

SEQ ID NO: 5090 - RNA, 20 nt, synthetic construct
  source 1..20: mol_type = other RNA
cgcccgcgcgctgcaacgaa

SEQ ID NO: 5091 - RNA, 20 nt, synthetic construct
  source 1..20: mol_type = other RNA
ctttcgttgcagcgcgcggg

SEQ ID NO: 5092 - RNA, 20 nt, synthetic construct
  source 1..20: mol_type = other RNA
cgcctttcgttgcagcgcgc

SEQ ID NO: 5093 - RNA, 20 nt, synthetic construct
  source 1..20: mol_type = other RNA
gcgcctttcgttgcagcgcg

SEQ ID NO: 5094 - RNA, 20 nt, synthetic construct
  source 1..20: mol_type = other RNA
gcaacgaaaggcgccgctca

SEQ ID NO: 5095 - RNA, 20 nt, synthetic construct
  source 1..20: mol_type = other RNA
cggctgggatgcaccttgag

SEQ ID NO: 5096 - RNA, 20 nt, synthetic construct
  source 1..20: mol_type = other RNA
gcatcccagccgcgccagag

SEQ ID NO: 5097 - RNA, 20 nt, synthetic construct
  source 1..20: mol_type = other RNA
gcggccgctctggcgcggct

SEQ ID NO: 5098 - RNA, 20 nt, synthetic construct
  source 1..20: mol_type = other RNA
ggcggccgctctggcgcggc

SEQ ID NO: 5099 - RNA, 20 nt, synthetic construct
  source 1..20: mol_type = other RNA
gggcggcggccgctctggcg

SEQ ID NO: 5100 - RNA, 20 nt, synthetic construct
  source 1..20: mol_type = other RNA
tgggcgggcggcggccgctc

SEQ ID NO: 5101 - RNA, 20 nt, synthetic construct
  source 1..20: mol_type = other RNA
ggtgggcggtgggcgggcgg

SEQ ID NO: 5102 - RNA, 20 nt, synthetic construct
  source 1..20: mol_type = other RNA
cccgcccaccgcccaccccc

SEQ ID NO: 5103 - RNA, 20 nt, synthetic construct
  source 1..20: mol_type = other RNA
gggggtgggcggtgggcggg

SEQ ID NO: 5104 - RNA, 20 nt, synthetic construct
  source 1..20: mol_type = other RNA
cccaccgcccacccccaggt

SEQ ID NO: 5105 - RNA, 20 nt, synthetic construct
  source 1..20: mol_type = other RNA
cctgggggtgggcggtgggc

SEQ ID NO: 5106 - RNA, 20 nt, synthetic construct
  source 1..20: mol_type = other RNA
caccgcccacccccaggtcg

SEQ ID NO: 5107 - RNA, 20 nt, synthetic construct
  source 1..20: mol_type = other RNA
ccgacctgggggtgggcggt

SEQ ID NO: 5108 - RNA, 20 nt, synthetic construct
  source 1..20: mol_type = other RNA
cccgacctgggggtgggcgg

SEQ ID NO: 5109 - RNA, 20 nt, synthetic construct
  source 1..20: mol_type = other RNA
agccccgacctgggggtggg

SEQ ID NO: 5110 - RNA, 20 nt, synthetic construct
  source 1..20: mol_type = other RNA
gggagccccgacctgggggt

SEQ ID NO: 5111 - RNA, 20 nt, synthetic construct
  source 1..20: mol_type = other RNA
cgggagccccgacctggggg

SEQ ID NO: 5112 - RNA, 20 nt, synthetic construct
  source 1..20: mol_type = other RNA
cgtcgggagccccgacctgg

SEQ ID NO: 5113 - RNA, 20 nt, synthetic construct
  source 1..20: mol_type = other RNA
gcgtcgggagccccgacctg

SEQ ID NO: 5114 - RNA, 20 nt, synthetic construct
  source 1..20: mol_type = other RNA
ggcgtcgggagccccgacct

SEQ ID NO: 5115 - RNA, 20 nt, synthetic construct
  source 1..20: mol_type = other RNA
gggcgtcgggagccccgacc

SEQ ID NO: 5116 - RNA, 20 nt, synthetic construct
  source 1..20: mol_type = other RNA
acgccccccgcccccgactc

SEQ ID NO: 5117 - RNA, 20 nt, synthetic construct
  source 1..20: mol_type = other RNA
cgccccccgcccccgactcc

SEQ ID NO: 5118 - RNA, 20 nt, synthetic construct
  source 1..20: mol_type = other RNA
gagtcgggggcggggggcgt

SEQ ID NO: 5119 - RNA, 20 nt, synthetic construct
  source 1..20: mol_type = other RNA
ccccgcccccgactccgggc

SEQ ID NO: 5120 - RNA, 20 nt, synthetic construct
  source 1..20: mol_type = other RNA
ggcccggagtcgggggcggg

SEQ ID NO: 5121 - RNA, 20 nt, synthetic construct
  source 1..20: mol_type = other RNA
cggcccggagtcgggggcgg

SEQ ID NO: 5122 - RNA, 20 nt, synthetic construct
  source 1..20: mol_type = other RNA
cccccgactccgggccggcc

SEQ ID NO: 5123 - RNA, 20 nt, synthetic construct
  source 1..20: mol_type = other RNA
gccggcccggagtcgggggc

SEQ ID NO: 5124 - RNA, 20 nt, synthetic construct
  source 1..20: mol_type = other RNA
ggccggcccggagtcggggg

SEQ ID NO: 5125 - RNA, 20 nt, synthetic construct
  source 1..20: mol_type = other RNA
cgactccgggccggccgggc

SEQ ID NO: 5126 - RNA, 20 nt, synthetic construct
  source 1..20: mol_type = other RNA
cccggccggcccggagtcgg

SEQ ID NO: 5127 - RNA, 20 nt, synthetic construct
  source 1..20: mol_type = other RNA
gcccggccggcccggagtcg

SEQ ID NO: 5128 - RNA, 20 nt, synthetic construct
  source 1..20: mol_type = other RNA
agcccggccggcccggagtc

SEQ ID NO: 5129 - RNA, 20 nt, synthetic construct
  source 1..20: mol_type = other RNA
cagcccggccggcccggagt

SEQ ID NO: 5130 - RNA, 20 nt, synthetic construct
  source 1..20: mol_type = other RNA
gccggccgggctggctgcag

SEQ ID NO: 5131 - RNA, 20 nt, synthetic construct
  source 1..20: mol_type = other RNA
tgcagccagcccggccggcc

SEQ ID NO: 5132 - RNA, 20 nt, synthetic construct
  source 1..20: mol_type = other RNA
gccgggctggctgcagcggc

SEQ ID NO: 5133 - RNA, 20 nt, synthetic construct
  source 1..20: mol_type = other RNA
gccgctgcagccagcccggc

SEQ ID NO: 5134 - RNA, 20 nt, synthetic construct
  source 1..20: mol_type = other RNA
gccggccgctgcagccagcc

SEQ ID NO: 5135 - RNA, 20 nt, synthetic construct
  source 1..20: mol_type = other RNA
cggcgcactcacccgctccc

SEQ ID NO: 5136 - RNA, 20 nt, synthetic construct
  source 1..20: mol_type = other RNA
cggggagcgggtgagtgcgc

SEQ ID NO: 5137 - RNA, 20 nt, synthetic construct
  source 1..20: mol_type = other RNA
ccgctccccggcttgcgcgc

SEQ ID NO: 5138 - RNA, 20 nt, synthetic construct
  source 1..20: mol_type = other RNA
ctgcgcgcaagccggggagc

SEQ ID NO: 5139 - RNA, 20 nt, synthetic construct
  source 1..20: mol_type = other RNA
cctgcgcgcaagccggggag

SEQ ID NO: 5140 - RNA, 20 nt, synthetic construct
  source 1..20: mol_type = other RNA
gtgtgcctgcgcgcaagccg

SEQ ID NO: 5141 - RNA, 20 nt, synthetic construct
  source 1..20: mol_type = other RNA
agtgtgcctgcgcgcaagcc

SEQ ID NO: 5142 - RNA, 20 nt, synthetic construct
  source 1..20: mol_type = other RNA
gagtgtgcctgcgcgcaagc

SEQ ID NO: 5143 - RNA, 20 nt, synthetic construct
  source 1..20: mol_type = other RNA
ggcggggggcggcggcggcg

SEQ ID NO: 5144 - RNA, 20 nt, synthetic construct
  source 1..20: mol_type = other RNA
ccgggggcggggggcggcgg

SEQ ID NO: 5145 - RNA, 20 nt, synthetic construct
  source 1..20: mol_type = other RNA
gggccgggggcggggggcgg

SEQ ID NO: 5146 - RNA, 20 nt, synthetic construct
  source 1..20: mol_type = other RNA
gcagggccgggggcgggggg

SEQ ID NO: 5147 - RNA, 20 nt, synthetic construct
  source 1..20: mol_type = other RNA
ggcgcagggccgggggcggg

SEQ ID NO: 5148 - RNA, 20 nt, synthetic construct
  source 1..20: mol_type = other RNA
gggcgcagggccgggggcgg

SEQ ID NO: 5149 - RNA, 20 nt, synthetic construct
  source 1..20: mol_type = other RNA
cgggcgcagggccgggggcg

SEQ ID NO: 5150 - RNA, 20 nt, synthetic construct
  source 1..20: mol_type = other RNA
gcgggcgcagggccgggggc

SEQ ID NO: 5151 - RNA, 20 nt, synthetic construct
  source 1..20: mol_type = other RNA
ggcgggcgcagggccggggg

SEQ ID NO: 5152 - RNA, 20 nt, synthetic construct
  source 1..20: mol_type = other RNA
aggggcgggcgcagggccgg

SEQ ID NO: 5153 - RNA, 20 nt, synthetic construct
  source 1..20: mol_type = other RNA
gaggggcgggcgcagggccg

SEQ ID NO: 5154 - RNA, 20 nt, synthetic construct
  source 1..20: mol_type = other RNA
ggaggggcgggcgcagggcc

SEQ ID NO: 5155 - RNA, 20 nt, synthetic construct
  source 1..20: mol_type = other RNA
aggaggggcgggcgcagggc

SEQ ID NO: 5156 - RNA, 20 nt, synthetic construct
  source 1..20: mol_type = other RNA
ggggaggaggggcgggcgca

SEQ ID NO: 5157 - RNA, 20 nt, synthetic construct
  source 1..20: mol_type = other RNA
aggggaggaggggcgggcgc

SEQ ID NO: 5158 - RNA, 20 nt, synthetic construct
  source 1..20: mol_type = other RNA
gcccctcctcccctccctcg

SEQ ID NO: 5159 - RNA, 20 nt, synthetic construct
  source 1..20: mol_type = other RNA
cgagggaggggaggaggggc

SEQ ID NO: 5160 - RNA, 20 nt, synthetic construct
  source 1..20: mol_type = other RNA
cctcctcccctccctcgcgg

SEQ ID NO: 5161 - RNA, 20 nt, synthetic construct
  source 1..20: mol_type = other RNA
gccgcgagggaggggaggag

SEQ ID NO: 5162 - RNA, 20 nt, synthetic construct
  source 1..20: mol_type = other RNA
cgccgcgagggaggggagga

SEQ ID NO: 5163 - RNA, 20 nt, synthetic construct
  source 1..20: mol_type = other RNA
tcccctccctcgcggcggcc

SEQ ID NO: 5164 - RNA, 20 nt, synthetic construct
  source 1..20: mol_type = other RNA
gggccgccgcgagggagggg

SEQ ID NO: 5165 - RNA, 20 nt, synthetic construct
  source 1..20: mol_type = other RNA
gccgggccgccgcgagggag

SEQ ID NO: 5166 - RNA, 20 nt, synthetic construct
  source 1..20: mol_type = other RNA
ggccgggccgccgcgaggga

SEQ ID NO: 5167 - RNA, 20 nt, synthetic construct
  source 1..20: mol_type = other RNA
gggccgggccgccgcgaggg

SEQ ID NO: 5168 - RNA, 20 nt, synthetic construct
  source 1..20: mol_type = other RNA
agcgggccgggccgccgcga

SEQ ID NO: 5169 - RNA, 20 nt, synthetic construct
  source 1..20: mol_type = other RNA
cagcgggccgggccgccgcg

SEQ ID NO: 5170 - RNA, 20 nt, synthetic construct
  source 1..20: mol_type = other RNA
ggcggctgcagcagcgggcc

SEQ ID NO: 5171 - RNA, 20 nt, synthetic construct
  source 1..20: mol_type = other RNA
cggcggctgcagcagcgggc

SEQ ID NO: 5172 - RNA, 20 nt, synthetic construct
  source 1..20: mol_type = other RNA
gcggcggcggctgcagcagc

SEQ ID NO: 5173 - RNA, 20 nt, synthetic construct
  source 1..20: mol_type = other RNA
ggcggcggcggctgcagcag

SEQ ID NO: 5174 - RNA, 20 nt, synthetic construct
  source 1..20: mol_type = other RNA
cgccgccgccgccgccgccg

SEQ ID NO: 5175 - RNA, 20 nt, synthetic construct
  source 1..20: mol_type = other RNA
ggcggcggcggcggcggcgg

SEQ ID NO: 5176 - RNA, 20 nt, synthetic construct
  source 1..20: mol_type = other RNA
cgcggcggcggcggcggcgg

SEQ ID NO: 5177 - RNA, 20 nt, synthetic construct
  source 1..20: mol_type = other RNA
caccgcggcggcggcggcgg

SEQ ID NO: 5178 - RNA, 20 nt, synthetic construct
  source 1..20: mol_type = other RNA
gagcaccgcggcggcggcgg

SEQ ID NO: 5179 - RNA, 20 nt, synthetic construct
  source 1..20: mol_type = other RNA
gcagagcaccgcggcggcgg

SEQ ID NO: 5180 - RNA, 20 nt, synthetic construct
  source 1..20: mol_type = other RNA
ggcgcagagcaccgcggcgg

SEQ ID NO: 5181 - RNA, 20 nt, synthetic construct
  source 1..20: mol_type = other RNA
gcgggcgcagagcaccgcgg

SEQ ID NO: 5182 - RNA, 20 nt, synthetic construct
  source 1..20: mol_type = other RNA
cgggcgggcgcagagcaccg

SEQ ID NO: 5183 - RNA, 20 nt, synthetic construct
  source 1..20: mol_type = other RNA
ccgcccgcctctttctcctc

SEQ ID NO: 5184 - RNA, 20 nt, synthetic construct
  source 1..20: mol_type = other RNA
cgcccgcctctttctcctcc

SEQ ID NO: 5185 - RNA, 20 nt, synthetic construct
  source 1..20: mol_type = other RNA
ccgcctctttctcctccggg

SEQ ID NO: 5186 - RNA, 20 nt, synthetic construct
  source 1..20: mol_type = other RNA
ccggaggagaaagaggcggg

SEQ ID NO: 5187 - RNA, 20 nt, synthetic construct
  source 1..20: mol_type = other RNA
ctcccggaggagaaagaggc

SEQ ID NO: 5188 - RNA, 20 nt, synthetic construct
  source 1..20: mol_type = other RNA
cctcccggaggagaaagagg

SEQ ID NO: 5189 - RNA, 20 nt, synthetic construct
  source 1..20: mol_type = other RNA
gcgcctcccggaggagaaag

SEQ ID NO: 5190 - RNA, 20 nt, synthetic construct
  source 1..20: mol_type = other RNA
ctccgggaggcgcgtgtgcg

SEQ ID NO: 5191 - RNA, 20 nt, synthetic construct
  source 1..20: mol_type = other RNA
tccgggaggcgcgtgtgcgc

SEQ ID NO: 5192 - RNA, 20 nt, synthetic construct
  source 1..20: mol_type = other RNA
cgcgcacacgcgcctcccgg

SEQ ID NO: 5193 - RNA, 20 nt, synthetic construct
  source 1..20: mol_type = other RNA
gaggcgcgtgtgcgcgggcg

SEQ ID NO: 5194 - RNA, 20 nt, synthetic construct
  source 1..20: mol_type = other RNA
gcccgcgcacacgcgcctcc

SEQ ID NO: 5195 - RNA, 20 nt, synthetic construct
  source 1..20: mol_type = other RNA
cgtgtgcgcgggcgaggccg

SEQ ID NO: 5196 - RNA, 20 nt, synthetic construct
  source 1..20: mol_type = other RNA
ctcacggtgcgcgcgcgcct

SEQ ID NO: 5197 - RNA, 20 nt, synthetic construct
  source 1..20: mol_type = other RNA
cgggcgcggcgcggggctca

SEQ ID NO: 5198 - RNA, 20 nt, synthetic construct
  source 1..20: mol_type = other RNA
cgcggggcgggcgcggcgcg

SEQ ID NO: 5199 - RNA, 20 nt, synthetic construct
  source 1..20: mol_type = other RNA
gcgcggggcgggcgcggcgc

SEQ ID NO: 5200 - RNA, 20 nt, synthetic construct
  source 1..20: mol_type = other RNA
cgcgcggggcgggcgcggcg

SEQ ID NO: 5201 - RNA, 20 nt, synthetic construct
  source 1..20: mol_type = other RNA
aggggcgcgcggggcgggcg

SEQ ID NO: 5202 - RNA, 20 nt, synthetic construct
  source 1..20: mol_type = other RNA
agtacaggggcgcgcggggc

SEQ ID NO: 5203 - RNA, 20 nt, synthetic construct
  source 1..20: mol_type = other RNA
gagtacaggggcgcgcgggg

SEQ ID NO: 5204 - RNA, 20 nt, synthetic construct
  source 1..20: mol_type = other RNA
ggggagtacaggggcgcgcg

SEQ ID NO: 5205 - RNA, 20 nt, synthetic construct
  source 1..20: mol_type = other RNA
cggggagtacaggggcgcgc

SEQ ID NO: 5206 - RNA, 20 nt, synthetic construct
  source 1..20: mol_type = other RNA
gcggggagtacaggggcgcg

SEQ ID NO: 5207 - RNA, 20 nt, synthetic construct
  source 1..20: mol_type = other RNA
gagcggcgcggggagtacag

SEQ ID NO: 5208 - RNA, 20 nt, synthetic construct
  source 1..20: mol_type = other RNA
ggagcggcgcggggagtaca

SEQ ID NO: 5209 - RNA, 20 nt, synthetic construct
  source 1..20: mol_type = other RNA
actccccgcgccgctcctcg

SEQ ID NO: 5210 - RNA, 20 nt, synthetic construct
  source 1..20: mol_type = other RNA
ggaccccgaggagcggcgcg

SEQ ID NO: 5211 - RNA, 20 nt, synthetic construct
  source 1..20: mol_type = other RNA
gggaccccgaggagcggcgc

SEQ ID NO: 5212 - RNA, 20 nt, synthetic construct
  source 1..20: mol_type = other RNA
cgggaccccgaggagcggcg

SEQ ID NO: 5213 - RNA, 20 nt, synthetic construct
  source 1..20: mol_type = other RNA
cgccgcgggaccccgaggag

SEQ ID NO: 5214 - RNA, 20 nt, synthetic construct
  source 1..20: mol_type = other RNA
cggggtcccgcggcgctcgc

SEQ ID NO: 5215 - RNA, 20 nt, synthetic construct
  source 1..20: mol_type = other RNA
gcgagcgccgcgggaccccg

SEQ ID NO: 5216 - RNA, 20 nt, synthetic construct
  source 1..20: mol_type = other RNA
gcgcggcctgcgagcgccgc

SEQ ID NO: 5217 - RNA, 20 nt, synthetic construct
  source 1..20: mol_type = other RNA
ggcgcggcctgcgagcgccg

SEQ ID NO: 5218 - RNA, 20 nt, synthetic construct
  source 1..20: mol_type = other RNA
agaggggcggcagggcggcg

SEQ ID NO: 5219 - RNA, 20 nt, synthetic construct
  source 1..20: mol_type = other RNA
gccctgccgcccctctctcg

SEQ ID NO: 5220 - RNA, 20 nt, synthetic construct
  source 1..20: mol_type = other RNA
acgagagaggggcggcaggg

SEQ ID NO: 5221 - RNA, 20 nt, synthetic construct
  source 1..20: mol_type = other RNA
gccacgagagaggggcggca

SEQ ID NO: 5222 - RNA, 20 nt, synthetic construct
  source 1..20: mol_type = other RNA
agccacgagagaggggcggc

SEQ ID NO: 5223 - RNA, 20 nt, synthetic construct
  source 1..20: mol_type = other RNA
cccctctctcgtggctttta

SEQ ID NO: 5224 - RNA, 20 nt, synthetic construct
  source 1..20: mol_type = other RNA
taaaagccacgagagagggg

SEQ ID NO: 5225 - RNA, 20 nt, synthetic construct
  source 1..20: mol_type = other RNA
ccgtaaaagccacgagagag

SEQ ID NO: 5226 - RNA, 20 nt, synthetic construct
  source 1..20: mol_type = other RNA
gccgtaaaagccacgagaga

SEQ ID NO: 5227 - RNA, 20 nt, synthetic construct
  source 1..20: mol_type = other RNA
ggccgtaaaagccacgagag

SEQ ID NO: 5228 - RNA, 20 nt, synthetic construct
  source 1..20: mol_type = other RNA
cgcccgcccctcagcagccc

SEQ ID NO: 5229 - RNA, 20 nt, synthetic construct
  source 1..20: mol_type = other RNA
gcccgcccctcagcagccct

SEQ ID NO: 5230 - RNA, 20 nt, synthetic construct
  source 1..20: mol_type = other RNA
cccgcccctcagcagccctg

SEQ ID NO: 5231 - RNA, 20 nt, synthetic construct
  source 1..20: mol_type = other RNA
agggctgctgaggggcgggc

SEQ ID NO: 5232 - RNA, 20 nt, synthetic construct
  source 1..20: mol_type = other RNA
cagggctgctgaggggcggg

SEQ ID NO: 5233 - RNA, 20 nt, synthetic construct
  source 1..20: mol_type = other RNA
ccccagggctgctgaggggc

SEQ ID NO: 5234 - RNA, 20 nt, synthetic construct
  source 1..20: mol_type = other RNA
accccagggctgctgagggg

SEQ ID NO: 5235 - RNA, 20 nt, synthetic construct
  source 1..20: mol_type = other RNA
ctcagcagccctggggtgcc

SEQ ID NO: 5236 - RNA, 20 nt, synthetic construct
  source 1..20: mol_type = other RNA
tcagcagccctggggtgccc

SEQ ID NO: 5237 - RNA, 20 nt, synthetic construct
  source 1..20: mol_type = other RNA
cagcagccctggggtgcccg

SEQ ID NO: 5238 - RNA, 20 nt, synthetic construct
  source 1..20: mol_type = other RNA
gggcaccccagggctgctga

SEQ ID NO: 5239 - RNA, 20 nt, synthetic construct
  source 1..20: mol_type = other RNA
cgggcaccccagggctgctg

SEQ ID NO: 5240 - RNA, 20 nt, synthetic construct
  source 1..20: mol_type = other RNA
cagccctggggtgcccgggg

SEQ ID NO: 5241 - RNA, 20 nt, synthetic construct
  source 1..20: mol_type = other RNA
gggccgccccgggcacccca

SEQ ID NO: 5242 - RNA, 20 nt, synthetic construct
  source 1..20: mol_type = other RNA
agggccgccccgggcacccc

SEQ ID NO: 5243 - RNA, 20 nt, synthetic construct
  source 1..20: mol_type = other RNA
gcccggggcggccctgcaag

SEQ ID NO: 5244 - RNA, 20 nt, synthetic construct
  source 1..20: mol_type = other RNA
cccggggcggccctgcaagc

SEQ ID NO: 5245 - RNA, 20 nt, synthetic construct
  source 1..20: mol_type = other RNA
cccgcttgcagggccgcccc

SEQ ID NO: 5246 - RNA, 20 nt, synthetic construct
  source 1..20: mol_type = other RNA
tcccgcttgcagggccgccc

SEQ ID NO: 5247 - RNA, 20 nt, synthetic construct
  source 1..20: mol_type = other RNA
gccctgcaagcgggagagag

SEQ ID NO: 5248 - RNA, 20 nt, synthetic construct
  source 1..20: mol_type = other RNA
gcaagcgggagagagcggcg

SEQ ID NO: 5249 - RNA, 20 nt, synthetic construct
  source 1..20: mol_type = other RNA
gccgctctctcccgcttgca

SEQ ID NO: 5250 - RNA, 20 nt, synthetic construct
  source 1..20: mol_type = other RNA
cgccgctctctcccgcttgc

SEQ ID NO: 5251 - RNA, 20 nt, synthetic construct
  source 1..20: mol_type = other RNA
agcgggagagagcggcgagg

SEQ ID NO: 5252 - RNA, 20 nt, synthetic construct
  source 1..20: mol_type = other RNA
gggagagagcggcgaggcgg

SEQ ID NO: 5253 - RNA, 20 nt, synthetic construct
  source 1..20: mol_type = other RNA
cgaggcggcggcgccgagtg

SEQ ID NO: 5254 - RNA, 20 nt, synthetic construct
  source 1..20: mol_type = other RNA
gaggcggcggcgccgagtgc

SEQ ID NO: 5255 - RNA, 20 nt, synthetic construct
  source 1..20: mol_type = other RNA
aggcggcggcgccgagtgcg

SEQ ID NO: 5256 - RNA, 20 nt, synthetic construct
  source 1..20: mol_type = other RNA
ggcggcggcgccgagtgcgg

SEQ ID NO: 5257 - RNA, 20 nt, synthetic construct
  source 1..20: mol_type = other RNA
gcggcggcgccgagtgcggg

SEQ ID NO: 5258 - RNA, 20 nt, synthetic construct
  source 1..20: mol_type = other RNA
gcgccgagtgcggggggatg

SEQ ID NO: 5259 - RNA, 20 nt, synthetic construct
  source 1..20: mol_type = other RNA
gctccgcatccccccgcact

SEQ ID NO: 5260 - RNA, 20 nt, synthetic construct
  source 1..20: mol_type = other RNA
gggggatgcggagccgtgcc

SEQ ID NO: 5261 - RNA, 20 nt, synthetic construct
  source 1..20: mol_type = other RNA
ggatgcgacagggccgggca

SEQ ID NO: 5262 - RNA, 20 nt, synthetic construct
  source 1..20: mol_type = other RNA
ccgagggatgcgacagggcc

SEQ ID NO: 5263 - RNA, 20 nt, synthetic construct
  source 1..20: mol_type = other RNA
gccgagggatgcgacagggc

SEQ ID NO: 5264 - RNA, 20 nt, synthetic construct
  source 1..20: mol_type = other RNA
ggcggccgagggatgcgaca

SEQ ID NO: 5265 - RNA, 20 nt, synthetic construct
  source 1..20: mol_type = other RNA
gggcggccgagggatgcgac

SEQ ID NO: 5266 - RNA, 20 nt, synthetic construct
  source 1..20: mol_type = other RNA
ctcggccgcccgcccgcgcc

SEQ ID NO: 5267 - RNA, 20 nt, synthetic construct
  source 1..20: mol_type = other RNA
gggcgcgggcgggcggccga

SEQ ID NO: 5268 - RNA, 20 nt, synthetic construct
  source 1..20: mol_type = other RNA
cgggcgcgggcgggcggccg

SEQ ID NO: 5269 - RNA, 20 nt, synthetic construct
  source 1..20: mol_type = other RNA
cgcccgcgcccggccccgcc

SEQ ID NO: 5270 - RNA, 20 nt, synthetic construct
  source 1..20: mol_type = other RNA
gggcggggccgggcgcgggc

SEQ ID NO: 5271 - RNA, 20 nt, synthetic construct
  source 1..20: mol_type = other RNA
cgggcggggccgggcgcggg

SEQ ID NO: 5272 - RNA, 20 nt, synthetic construct
  source 1..20: mol_type = other RNA
ggccgggcggggccgggcgc

SEQ ID NO: 5273 - RNA, 20 nt, synthetic construct
  source 1..20: mol_type = other RNA
aggccgggcggggccgggcg

SEQ ID NO: 5274 - RNA, 20 nt, synthetic construct
  source 1..20: mol_type = other RNA
cggccccgcccggccttgcc

SEQ ID NO: 5275 - RNA, 20 nt, synthetic construct
  source 1..20: mol_type = other RNA
ggccccgcccggccttgccc

SEQ ID NO: 5276 - RNA, 20 nt, synthetic construct
  source 1..20: mol_type = other RNA
gggcaaggccgggcggggcc

SEQ ID NO: 5277 - RNA, 20 nt, synthetic construct
  source 1..20: mol_type = other RNA
cgggcaaggccgggcggggc

SEQ ID NO: 5278 - RNA, 20 nt, synthetic construct
  source 1..20: mol_type = other RNA
agcccgggcaaggccgggcg

SEQ ID NO: 5279 - RNA, 20 nt, synthetic construct
  source 1..20: mol_type = other RNA
cagcccgggcaaggccgggc

SEQ ID NO: 5280 - RNA, 20 nt, synthetic construct
  source 1..20: mol_type = other RNA
gcagcccgggcaaggccggg

SEQ ID NO: 5281 - RNA, 20 nt, synthetic construct
  source 1..20: mol_type = other RNA
cgtgcagcccgggcaaggcc

SEQ ID NO: 5282 - RNA, 20 nt, synthetic construct
  source 1..20: mol_type = other RNA
gcgtgcagcccgggcaaggc

SEQ ID NO: 5283 - RNA, 20 nt, synthetic construct
  source 1..20: mol_type = other RNA
aagtgcgtgcagcccgggca

SEQ ID NO: 5284 - RNA, 20 nt, synthetic construct
  source 1..20: mol_type = other RNA
ggctgcacgcacttctcccg

SEQ ID NO: 5285 - RNA, 20 nt, synthetic construct
  source 1..20: mol_type = other RNA
gggagaagtgcgtgcagccc

SEQ ID NO: 5286 - RNA, 20 nt, synthetic construct
  source 1..20: mol_type = other RNA
cgggagaagtgcgtgcagcc

SEQ ID NO: 5287 - RNA, 20 nt, synthetic construct
  source 1..20: mol_type = other RNA
tcaagtggattctgggccgc

SEQ ID NO: 5288 - RNA, 20 nt, synthetic construct
  source 1..20: mol_type = other RNA
gtcaagtggattctgggccg

SEQ ID NO: 5289 - RNA, 20 nt, synthetic construct
  source 1..20: mol_type = other RNA
cagaatccacttgaccctgc

SEQ ID NO: 5290 - RNA, 20 nt, synthetic construct
  source 1..20: mol_type = other RNA
agaatccacttgaccctgct

SEQ ID NO: 5291 - RNA, 20 nt, synthetic construct
  source 1..20: mol_type = other RNA
agcagggtcaagtggattct

SEQ ID NO: 5292 - RNA, 20 nt, synthetic construct
  source 1..20: mol_type = other RNA
cagcagggtcaagtggattc

SEQ ID NO: 5293 - RNA, 20 nt, synthetic construct
  source 1..20: mol_type = other RNA
gagcgcccagcagggtcaag

SEQ ID NO: 5294 - RNA, 20 nt, synthetic construct
  source 1..20: mol_type = other RNA
gaccctgctgggcgctcccg

SEQ ID NO: 5295 - RNA, 20 nt, synthetic construct
  source 1..20: mol_type = other RNA
accctgctgggcgctcccgc

SEQ ID NO: 5296 - RNA, 20 nt, synthetic construct
  source 1..20: mol_type = other RNA
ctgctgggcgctcccgcggg

SEQ ID NO: 5297 - RNA, 20 nt, synthetic construct
  source 1..20: mol_type = other RNA
gcccgcgggagcgcccagca

SEQ ID NO: 5298 - RNA, 20 nt, synthetic construct
  source 1..20: mol_type = other RNA
cgcccgcgggagcgcccagc

SEQ ID NO: 5299 - RNA, 20 nt, synthetic construct
  source 1..20: mol_type = other RNA
gctcccgcgggcggcggacc

SEQ ID NO: 5300 - RNA, 20 nt, synthetic construct
  source 1..20: mol_type = other RNA
ctcccgcgggcggcggaccc

SEQ ID NO: 5301 - RNA, 20 nt, synthetic construct
  source 1..20: mol_type = other RNA
ccgcgggcggcggacccggg

SEQ ID NO: 5302 - RNA, 20 nt, synthetic construct
  source 1..20: mol_type = other RNA
cgcgggcggcggacccgggt

SEQ ID NO: 5303 - RNA, 20 nt, synthetic construct
  source 1..20: mol_type = other RNA
cacccgggtccgccgcccgc

SEQ ID NO: 5304 - RNA, 20 nt, synthetic construct
  source 1..20: mol_type = other RNA
ccacccgggtccgccgcccg

SEQ ID NO: 5305 - RNA, 20 nt, synthetic construct
  source 1..20: mol_type = other RNA
gcggcggacccgggtgggtg

SEQ ID NO: 5306 - RNA, 20 nt, synthetic construct
  source 1..20: mol_type = other RNA
cggcggacccgggtgggtgc

SEQ ID NO: 5307 - RNA, 20 nt, synthetic construct
  source 1..20: mol_type = other RNA
ggcggacccgggtgggtgcg

SEQ ID NO: 5308 - RNA, 20 nt, synthetic construct
  source 1..20: mol_type = other RNA
gcggacccgggtgggtgcgg

SEQ ID NO: 5309 - RNA, 20 nt, synthetic construct
  source 1..20: mol_type = other RNA
gaattcccccgcacccaccc

SEQ ID NO: 5310 - RNA, 20 nt, synthetic construct
  source 1..20: mol_type = other RNA
ggaattcccccgcacccacc

SEQ ID NO: 5311 - RNA, 20 nt, synthetic construct
  source 1..20: mol_type = other RNA
ggggaattccccggccgccc

SEQ ID NO: 5312 - RNA, 20 nt, synthetic construct
  source 1..20: mol_type = other RNA
attccccggccgcccaggcg

SEQ ID NO: 5313 - RNA, 20 nt, synthetic construct
  source 1..20: mol_type = other RNA
ttccccggccgcccaggcgc

SEQ ID NO: 5314 - RNA, 20 nt, synthetic construct
  source 1..20: mol_type = other RNA
tccccggccgcccaggcgcg

SEQ ID NO: 5315 - RNA, 20 nt, synthetic construct
  source 1..20: mol_type = other RNA
tccccgcgcctgggcggccg

SEQ ID NO: 5316 - RNA, 20 nt, synthetic construct
  source 1..20: mol_type = other RNA
ctccccgcgcctgggcggcc

SEQ ID NO: 5317 - RNA, 20 nt, synthetic construct
  source 1..20: mol_type = other RNA
tctccccgcgcctgggcggc

SEQ ID NO: 5318 - RNA, 20 nt, synthetic construct
  source 1..20: mol_type = other RNA
tcactctccccgcgcctggg

SEQ ID NO: 5319 - RNA, 20 nt, synthetic construct
  source 1..20: mol_type = other RNA
agctcactctccccgcgcct

SEQ ID NO: 5320 - RNA, 20 nt, synthetic construct
  source 1..20: mol_type = other RNA
cagctcactctccccgcgcc

SEQ ID NO: 5321 - RNA, 20 nt, synthetic construct
  source 1..20: mol_type = other RNA
gtttggggcgctgctgcggg

SEQ ID NO: 5322 - RNA, 20 nt, synthetic construct
  source 1..20: mol_type = other RNA
tttgtttggggcgctgctgc

SEQ ID NO: 5323 - RNA, 20 nt, synthetic construct
  source 1..20: mol_type = other RNA
gtttgtttggggcgctgctg

SEQ ID NO: 5324 - RNA, 20 nt, synthetic construct
  source 1..20: mol_type = other RNA
cgccccaaacaaaccgttta

SEQ ID NO: 5325 - RNA, 20 nt, synthetic construct
  source 1..20: mol_type = other RNA
aacaaaccgtttaaggtctc

SEQ ID NO: 5326 - RNA, 20 nt, synthetic construct
  source 1..20: mol_type = other RNA
agaccttaaacggtttgttt

SEQ ID NO: 5327 - RNA, 20 nt, synthetic construct
  source 1..20: mol_type = other RNA
gagaccttaaacggtttgtt

SEQ ID NO: 5328 - RNA, 20 nt, synthetic construct
  source 1..20: mol_type = other RNA
cgggctccagagaccttaaa

SEQ ID NO: 5329 - RNA, 20 nt, synthetic construct
  source 1..20: mol_type = other RNA
gcaagttcagcgaaataaag

SEQ ID NO: 5330 - RNA, 20 nt, synthetic construct
  source 1..20: mol_type = other RNA
ctttatttcgctgaacttgc

SEQ ID NO: 5331 - RNA, 20 nt, synthetic construct
  source 1..20: mol_type = other RNA
gctttatttcgctgaacttg

SEQ ID NO: 5332 - RNA, 20 nt, synthetic construct
  source 1..20: mol_type = other RNA
agcgaaataaagcggcggcg

SEQ ID NO: 5333 - RNA, 20 nt, synthetic construct
  source 1..20: mol_type = other RNA
gaaataaagcggcggcgcgg

SEQ ID NO: 5334 - RNA, 20 nt, synthetic construct
  source 1..20: mol_type = other RNA
cggaggaaacctcttccacc

SEQ ID NO: 5335 - RNA, 20 nt, synthetic construct
  source 1..20: mol_type = other RNA
agagcaggtccgggtggaag

SEQ ID NO: 5336 - RNA, 20 nt, synthetic construct
  source 1..20: mol_type = other RNA
cccggacctgctctccgttg

SEQ ID NO: 5337 - RNA, 20 nt, synthetic construct
  source 1..20: mol_type = other RNA
caacggagagcaggtccggg

SEQ ID NO: 5338 - RNA, 20 nt, synthetic construct
  source 1..20: mol_type = other RNA
ccgcaacggagagcaggtcc

SEQ ID NO: 5339 - RNA, 20 nt, synthetic construct
  source 1..20: mol_type = other RNA
accgcaacggagagcaggtc

SEQ ID NO: 5340 - RNA, 20 nt, synthetic construct
  source 1..20: mol_type = other RNA
gccaaaccgcaacggagagc

SEQ ID NO: 5341 - RNA, 20 nt, synthetic construct
  source 1..20: mol_type = other RNA
cgttgcggtttggcctccag

SEQ ID NO: 5342 - RNA, 20 nt, synthetic construct
  source 1..20: mol_type = other RNA
tgcggtttggcctccagtgg

SEQ ID NO: 5343 - RNA, 20 nt, synthetic construct
  source 1..20: mol_type = other RNA
cactggaggccaaaccgcaa

SEQ ID NO: 5344 - RNA, 20 nt, synthetic construct
  source 1..20: mol_type = other RNA
gtgggtgggaccaccactgg

SEQ ID NO: 5345 - RNA, 20 nt, synthetic construct
  source 1..20: mol_type = other RNA
agggtgggtgggaccaccac

SEQ ID NO: 5346 - RNA, 20 nt, synthetic construct
  source 1..20: mol_type = other RNA
ggtcccacccaccctctagc

SEQ ID NO: 5347 - RNA, 20 nt, synthetic construct
  source 1..20: mol_type = other RNA
tggccagctagagggtgggt

SEQ ID NO: 5348 - RNA, 20 nt, synthetic construct
  source 1..20: mol_type = other RNA
ctggccagctagagggtggg

SEQ ID NO: 5349 - RNA, 20 nt, synthetic construct
  source 1..20: mol_type = other RNA
accctctagctggccagccc

SEQ ID NO: 5350 - RNA, 20 nt, synthetic construct
  source 1..20: mol_type = other RNA
gggctggccagctagagggt

SEQ ID NO: 5351 - RNA, 20 nt, synthetic construct
  source 1..20: mol_type = other RNA
agggctggccagctagaggg

SEQ ID NO: 5352 - RNA, 20 nt, synthetic construct
  source 1..20: mol_type = other RNA
tccagggctggccagctaga

SEQ ID NO: 5353 - RNA, 20 nt, synthetic construct
  source 1..20: mol_type = other RNA
ttccagggctggccagctag

SEQ ID NO: 5354 - RNA, 20 nt, synthetic construct
  source 1..20: mol_type = other RNA
aggaggttggtttccagggc

SEQ ID NO: 5355 - RNA, 20 nt, synthetic construct
  source 1..20: mol_type = other RNA
agaaaggaggttggtttcca

SEQ ID NO: 5356 - RNA, 20 nt, synthetic construct
  source 1..20: mol_type = other RNA
aagaaaggaggttggtttcc

SEQ ID NO: 5357 - RNA, 20 nt, synthetic construct
  source 1..20: mol_type = other RNA
gaaataaaaagaaaggaggt

SEQ ID NO: 5358 - RNA, 20 nt, synthetic construct
  source 1..20: mol_type = other RNA
cctttctttttatttctcac

SEQ ID NO: 5359 - RNA, 20 nt, synthetic construct
  source 1..20: mol_type = other RNA
ctttctttttatttctcacc

SEQ ID NO: 5360 - RNA, 20 nt, synthetic construct
  source 1..20: mol_type = other RNA
gtgagaaataaaaagaaagg

SEQ ID NO: 5361 - RNA, 20 nt, synthetic construct
  source 1..20: mol_type = other RNA
ctttttatttctcaccggga

SEQ ID NO: 5362 - RNA, 20 nt, synthetic construct
  source 1..20: mol_type = other RNA
tttttatttctcaccgggaa

SEQ ID NO: 5363 - RNA, 20 nt, synthetic construct
  source 1..20: mol_type = other RNA
ttttatttctcaccgggaag

SEQ ID NO: 5364 - RNA, 20 nt, synthetic construct
  source 1..20: mol_type = other RNA
tttatttctcaccgggaagg

SEQ ID NO: 5365 - RNA, 20 nt, synthetic construct
  source 1..20: mol_type = other RNA
caccgggaagggggacaaac

SEQ ID NO: 5366 - RNA, 20 nt, synthetic construct
  source 1..20: mol_type = other RNA
ggccagtttgtcccccttcc

SEQ ID NO: 5367 - RNA, 20 nt, synthetic construct
  source 1..20: mol_type = other RNA
agggggacaaactggcctct

SEQ ID NO: 5368 - RNA, 20 nt, synthetic construct
  source 1..20: mol_type = other RNA
agtttgaagtcgacacccag

SEQ ID NO: 5369 - RNA, 20 nt, synthetic construct
  source 1..20: mol_type = other RNA
tcaaacttgccgcccgtctc

SEQ ID NO: 5370 - RNA, 20 nt, synthetic construct
  source 1..20: mol_type = other RNA
cttgccgcccgtctccggtc

SEQ ID NO: 5371 - RNA, 20 nt, synthetic construct
  source 1..20: mol_type = other RNA
cgcccgtctccggtctggaa

SEQ ID NO: 5372 - RNA, 20 nt, synthetic construct
  source 1..20: mol_type = other RNA
ctttccagaccggagacggg

SEQ ID NO: 5373 - RNA, 20 nt, synthetic construct
  source 1..20: mol_type = other RNA
tgcctttccagaccggagac

SEQ ID NO: 5374 - RNA, 20 nt, synthetic construct
  source 1..20: mol_type = other RNA
ctgcctttccagaccggaga

SEQ ID NO: 5375 - RNA, 20 nt, synthetic construct
  source 1..20: mol_type = other RNA
gatcacctgcctttccagac

SEQ ID NO: 5376 - RNA, 20 nt, synthetic construct
  source 1..20: mol_type = other RNA
aaggcaggtgatcagctaga

SEQ ID NO: 5377 - RNA, 20 nt, synthetic construct
  source 1..20: mol_type = other RNA
aggcaggtgatcagctagaa

SEQ ID NO: 5378 - RNA, 20 nt, synthetic construct
  source 1..20: mol_type = other RNA
gggtgataagagtatcatcg

SEQ ID NO: 5379 - RNA, 20 nt, synthetic construct
  source 1..20: mol_type = other RNA
ggagattattattactcttt

SEQ ID NO: 5380 - RNA, 20 nt, synthetic construct
  source 1..20: mol_type = other RNA
aagagctgtctttacaatga

SEQ ID NO: 5381 - RNA, 20 nt, synthetic construct
  source 1..20: mol_type = other RNA
gaagagctgtctttacaatg

SEQ ID NO: 5382 - RNA, 20 nt, synthetic construct
  source 1..20: mol_type = other RNA
gtaaagacagctcttccccc

SEQ ID NO: 5383 - RNA, 20 nt, synthetic construct
  source 1..20: mol_type = other RNA
gtctaaaaaagtaagccagg

SEQ ID NO: 5384 - RNA, 20 nt, synthetic construct
  source 1..20: mol_type = other RNA
tgtctaaaaaagtaagccag

SEQ ID NO: 5385 - RNA, 20 nt, synthetic construct
  source 1..20: mol_type = other RNA
atgtctaaaaaagtaagcca

SEQ ID NO: 5386 - RNA, 20 nt, synthetic construct
  source 1..20: mol_type = other RNA
catgtctaaaaaagtaagcc

SEQ ID NO: 5387 - RNA, 20 nt, synthetic construct
  source 1..20: mol_type = other RNA
gagaagcgcatgtctccatc

SEQ ID NO: 5388 - RNA, 20 nt, synthetic construct
  source 1..20: mol_type = other RNA
agaagcgcatgtctccatca

SEQ ID NO: 5389 - RNA, 20 nt, synthetic construct
  source 1..20: mol_type = other RNA
aagcagaggtagggccctga

SEQ ID NO: 5390 - RNA, 20 nt, synthetic construct
  source 1..20: mol_type = other RNA
tacctctgcttctccacagt

SEQ ID NO: 5391 - RNA, 20 nt, synthetic construct
  source 1..20: mol_type = other RNA
actgtggagaagcagaggta

SEQ ID NO: 5392 - RNA, 20 nt, synthetic construct
  source 1..20: mol_type = other RNA
aactgtggagaagcagaggt

SEQ ID NO: 5393 - RNA, 20 nt, synthetic construct
  source 1..20: mol_type = other RNA
ggccaactgtggagaagcag

SEQ ID NO: 5394 - RNA, 20 nt, synthetic construct
  source 1..20: mol_type = other RNA
ctccacagttggcctagaac

SEQ ID NO: 5395 - RNA, 20 nt, synthetic construct
  source 1..20: mol_type = other RNA
ttccggttctaggccaactg

SEQ ID NO: 5396 - RNA, 20 nt, synthetic construct
  source 1..20: mol_type = other RNA
tagaaccggaagcccctcca

SEQ ID NO: 5397 - RNA, 20 nt, synthetic construct
  source 1..20: mol_type = other RNA
ttggaggggcttccggttct

SEQ ID NO: 5398 - RNA, 20 nt, synthetic construct
  source 1..20: mol_type = other RNA
gggggccttggaggggcttc

SEQ ID NO: 5399 - RNA, 20 nt, synthetic construct
  source 1..20: mol_type = other RNA
agagtcagggggccttggag

SEQ ID NO: 5400 - RNA, 20 nt, synthetic construct
  source 1..20: mol_type = other RNA
gagagtcagggggccttgga

SEQ ID NO: 5401 - RNA, 20 nt, synthetic construct
  source 1..20: mol_type = other RNA
ggagagtcagggggccttgg

SEQ ID NO: 5402 - RNA, 20 nt, synthetic construct
  source 1..20: mol_type = other RNA
tcaggagagtcagggggcct

SEQ ID NO: 5403 - RNA, 20 nt, synthetic construct
  source 1..20: mol_type = other RNA
ccctgactctcctgacctct

SEQ ID NO: 5404 - RNA, 20 nt, synthetic construct
  source 1..20: mol_type = other RNA
aagaggtcaggagagtcagg

SEQ ID NO: 5405 - RNA, 20 nt, synthetic construct
  source 1..20: mol_type = other RNA
caagaggtcaggagagtcag

SEQ ID NO: 5406 - RNA, 20 nt, synthetic construct
  source 1..20: mol_type = other RNA
ccaagaggtcaggagagtca

SEQ ID NO: 5407 - RNA, 20 nt, synthetic construct
  source 1..20: mol_type = other RNA
gccaagaggtcaggagagtc

SEQ ID NO: 5408 - RNA, 20 nt, synthetic construct
  source 1..20: mol_type = other RNA
tgacctcttggccacagctc

SEQ ID NO: 5409 - RNA, 20 nt, synthetic construct
  source 1..20: mol_type = other RNA
ggagctgtggccaagaggtc

SEQ ID NO: 5410 - RNA, 20 nt, synthetic construct
  source 1..20: mol_type = other RNA
aatccggagctgtggccaag

SEQ ID NO: 5411 - RNA, 20 nt, synthetic construct
  source 1..20: mol_type = other RNA
cacagctccggattctcacc

SEQ ID NO: 5412 - RNA, 20 nt, synthetic construct
  source 1..20: mol_type = other RNA
acagctccggattctcacca

SEQ ID NO: 5413 - RNA, 20 nt, synthetic construct
  source 1..20: mol_type = other RNA
ctggtgagaatccggagctg

SEQ ID NO: 5414 - RNA, 20 nt, synthetic construct
  source 1..20: mol_type = other RNA
gggaatccctggtgagaatc

SEQ ID NO: 5415 - RNA, 20 nt, synthetic construct
  source 1..20: mol_type = other RNA
taggaattctggggaatccc

SEQ ID NO: 5416 - RNA, 20 nt, synthetic construct
  source 1..20: mol_type = other RNA
gctgctctctaggaattctg

SEQ ID NO: 5417 - RNA, 20 nt, synthetic construct
  source 1..20: mol_type = other RNA
agctgctctctaggaattct

SEQ ID NO: 5418 - RNA, 20 nt, synthetic construct
  source 1..20: mol_type = other RNA
gagctgctctctaggaattc

SEQ ID NO: 5419 - RNA, 20 nt, synthetic construct
  source 1..20: mol_type = other RNA
agggctctgagctgctctct

SEQ ID NO: 5420 - RNA, 20 nt, synthetic construct
  source 1..20: mol_type = other RNA
cgtggtgaggcacaactgca

SEQ ID NO: 5421 - RNA, 20 nt, synthetic construct
  source 1..20: mol_type = other RNA
gcgtggtgaggcacaactgc

SEQ ID NO: 5422 - RNA, 20 nt, synthetic construct
  source 1..20: mol_type = other RNA
gaggtttggttcgcgtggtg

SEQ ID NO: 5423 - RNA, 20 nt, synthetic construct
  source 1..20: mol_type = other RNA
agtgcgaggtttggttcgcg

SEQ ID NO: 5424 - RNA, 20 nt, synthetic construct
  source 1..20: mol_type = other RNA
acctcgcactccccgccaaa

SEQ ID NO: 5425 - RNA, 20 nt, synthetic construct
  source 1..20: mol_type = other RNA
ttggcggggagtgcgaggtt

SEQ ID NO: 5426 - RNA, 20 nt, synthetic construct
  source 1..20: mol_type = other RNA
cccttttggcggggagtgcg

SEQ ID NO: 5427 - RNA, 20 nt, synthetic construct
  source 1..20: mol_type = other RNA
gaagggactcccttttggcg

SEQ ID NO: 5428 - RNA, 20 nt, synthetic construct
  source 1..20: mol_type = other RNA
ggaagggactcccttttggc

SEQ ID NO: 5429 - RNA, 20 nt, synthetic construct
  source 1..20: mol_type = other RNA
tggaagggactcccttttgg

SEQ ID NO: 5430 - RNA, 20 nt, synthetic construct
  source 1..20: mol_type = other RNA
tgctggaagggactcccttt

SEQ ID NO: 5431 - RNA, 20 nt, synthetic construct
  source 1..20: mol_type = other RNA
caaaggggagagtgctggaa

SEQ ID NO: 5432 - RNA, 20 nt, synthetic construct
  source 1..20: mol_type = other RNA
acaaaggggagagtgctgga

SEQ ID NO: 5433 - RNA, 20 nt, synthetic construct
  source 1..20: mol_type = other RNA
aggaacaaaggggagagtgc

SEQ ID NO: 5434 - RNA, 20 nt, synthetic construct
  source 1..20: mol_type = other RNA
ctcccctttgttcctttttc

SEQ ID NO: 5435 - RNA, 20 nt, synthetic construct
  source 1..20: mol_type = other RNA
tcccctttgttcctttttct

SEQ ID NO: 5436 - RNA, 20 nt, synthetic construct
  source 1..20: mol_type = other RNA
gcccagaaaaaggaacaaag

SEQ ID NO: 5437 - RNA, 20 nt, synthetic construct
  source 1..20: mol_type = other RNA
tgcccagaaaaaggaacaaa

SEQ ID NO: 5438 - RNA, 20 nt, synthetic construct
  source 1..20: mol_type = other RNA
ttgcccagaaaaaggaacaa

SEQ ID NO: 5439 - RNA, 20 nt, synthetic construct
  source 1..20: mol_type = other RNA
agcggttcttgcccagaaaa

SEQ ID NO: 5440 - RNA, 20 nt, synthetic construct
  source 1..20: mol_type = other RNA
tctgggcaagaaccgctgac

SEQ ID NO: 5441 - RNA, 20 nt, synthetic construct
  source 1..20: mol_type = other RNA
ctgggcaagaaccgctgact

SEQ ID NO: 5442 - RNA, 20 nt, synthetic construct
  source 1..20: mol_type = other RNA
tgggcaagaaccgctgactg

SEQ ID NO: 5443 - RNA, 20 nt, synthetic construct
  source 1..20: mol_type = other RNA
tttctggcagccccagtcag

SEQ ID NO: 5444 - RNA, 20 nt, synthetic construct
  source 1..20: mol_type = other RNA
gctgccagaaatgtaaaccc

SEQ ID NO: 5445 - RNA, 20 nt, synthetic construct
  source 1..20: mol_type = other RNA
ctgccagaaatgtaaaccct

SEQ ID NO: 5446 - RNA, 20 nt, synthetic construct
  source 1..20: mol_type = other RNA
gcacccagggtttacatttc

SEQ ID NO: 5447 - RNA, 20 nt, synthetic construct
  source 1..20: mol_type = other RNA
taaaccctgggtgcaagtga

SEQ ID NO: 5448 - RNA, 20 nt, synthetic construct
  source 1..20: mol_type = other RNA
aaaccctgggtgcaagtgac

SEQ ID NO: 5449 - RNA, 20 nt, synthetic construct
  source 1..20: mol_type = other RNA
gatcccgtcacttgcaccca

SEQ ID NO: 5450 - RNA, 20 nt, synthetic construct
  source 1..20: mol_type = other RNA
ggatcccgtcacttgcaccc

SEQ ID NO: 5451 - RNA, 20 nt, synthetic construct
  source 1..20: mol_type = other RNA
ctcttcggcttgacgctgga

SEQ ID NO: 5452 - RNA, 20 nt, synthetic construct
  source 1..20: mol_type = other RNA
actcttcggcttgacgctgg

SEQ ID NO: 5453 - RNA, 20 nt, synthetic construct
  source 1..20: mol_type = other RNA
atgactcttcggcttgacgc

SEQ ID NO: 5454 - RNA, 20 nt, synthetic construct
  source 1..20: mol_type = other RNA
gaggtgagaggatgactctt

SEQ ID NO: 5455 - RNA, 20 nt, synthetic construct
  source 1..20: mol_type = other RNA
tcggaggtgggtgaggtgag

SEQ ID NO: 5456 - RNA, 20 nt, synthetic construct
  source 1..20: mol_type = other RNA
acctcacccacctccgaatg

SEQ ID NO: 5457 - RNA, 20 nt, synthetic construct
  source 1..20: mol_type = other RNA
tcctcattcggaggtgggtg

SEQ ID NO: 5458 - RNA, 20 nt, synthetic construct
  source 1..20: mol_type = other RNA
gttaatcctcattcggaggt

SEQ ID NO: 5459 - RNA, 20 nt, synthetic construct
  source 1..20: mol_type = other RNA
tgttaatcctcattcggagg

SEQ ID NO: 5460 - RNA, 20 nt, synthetic construct
  source 1..20: mol_type = other RNA
gtttgttaatcctcattcgg

SEQ ID NO: 5461 - RNA, 20 nt, synthetic construct
  source 1..20: mol_type = other RNA
tgagtttgttaatcctcatt

SEQ ID NO: 5462 - RNA, 20 nt, synthetic construct
  source 1..20: mol_type = other RNA
aggattaacaaactcaattc

SEQ ID NO: 5463 - RNA, 20 nt, synthetic construct
  source 1..20: mol_type = other RNA
acaaactcaattcaggacac

SEQ ID NO: 5464 - RNA, 20 nt, synthetic construct
  source 1..20: mol_type = other RNA
gacacaggtagaagaccaaa

SEQ ID NO: 5465 - RNA, 20 nt, synthetic construct
  source 1..20: mol_type = other RNA
aagaagtctcattggccttt

SEQ ID NO: 5466 - RNA, 20 nt, synthetic construct
  source 1..20: mol_type = other RNA
aaataggaaagaagtctcat

SEQ ID NO: 5467 - RNA, 20 nt, synthetic construct
  source 1..20: mol_type = other RNA
acttctttcctatttgagat

SEQ ID NO: 5468 - RNA, 20 nt, synthetic construct
  source 1..20: mol_type = other RNA
tctcaaatccgatctcaaat

SEQ ID NO: 5469 - RNA, 20 nt, synthetic construct
  source 1..20: mol_type = other RNA
ggatttgagaatgctcagcc

SEQ ID NO: 5470 - RNA, 20 nt, synthetic construct
  source 1..20: mol_type = other RNA
gctgggggaagaagggagcc

SEQ ID NO: 5471 - RNA, 20 nt, synthetic construct
  source 1..20: mol_type = other RNA
attcagagctgggggaagaa

SEQ ID NO: 5472 - RNA, 20 nt, synthetic construct
  source 1..20: mol_type = other RNA
gattcagagctgggggaaga

SEQ ID NO: 5473 - RNA, 20 nt, synthetic construct
  source 1..20: mol_type = other RNA
aaggattgattcagagctgg

SEQ ID NO: 5474 - RNA, 20 nt, synthetic construct
  source 1..20: mol_type = other RNA
aaaggattgattcagagctg

SEQ ID NO: 5475 - RNA, 20 nt, synthetic construct
  source 1..20: mol_type = other RNA
gaaaggattgattcagagct

SEQ ID NO: 5476 - RNA, 20 nt, synthetic construct
  source 1..20: mol_type = other RNA
agaaaggattgattcagagc

SEQ ID NO: 5477 - RNA, 20 nt, synthetic construct
  source 1..20: mol_type = other RNA
ttatggatgctaatgaagaa

SEQ ID NO: 5478 - RNA, 20 nt, synthetic construct
  source 1..20: mol_type = other RNA
tacattttgcacattagtta

SEQ ID NO: 5479 - RNA, 20 nt, synthetic construct
  source 1..20: mol_type = other RNA
acgctaaattaagacagagt

SEQ ID NO: 5480 - RNA, 20 nt, synthetic construct
  source 1..20: mol_type = other RNA
ctaatgagaggggtttttga

SEQ ID NO: 5481 - RNA, 20 nt, synthetic construct
  source 1..20: mol_type = other RNA
gctaatgagaggggtttttg

SEQ ID NO: 5482 - RNA, 20 nt, synthetic construct
  source 1..20: mol_type = other RNA
aaacccctctcattagctga

SEQ ID NO: 5483 - RNA, 20 nt, synthetic construct
  source 1..20: mol_type = other RNA
ctaccttcagctaatgagag

SEQ ID NO: 5484 - RNA, 20 nt, synthetic construct
  source 1..20: mol_type = other RNA
gctaccttcagctaatgaga

SEQ ID NO: 5485 - RNA, 20 nt, synthetic construct
  source 1..20: mol_type = other RNA
tgctaccttcagctaatgag

SEQ ID NO: 5486 - RNA, 20 nt, synthetic construct
  source 1..20: mol_type = other RNA
tagcaagtagcaagaagatt

SEQ ID NO: 5487 - RNA, 20 nt, synthetic construct
  source 1..20: mol_type = other RNA
aacatagagaatatgaatat

SEQ ID NO: 5488 - RNA, 20 nt, synthetic construct
  source 1..20: mol_type = other RNA
atgaatataggaaaaagtac

SEQ ID NO: 5489 - RNA, 20 nt, synthetic construct
  source 1..20: mol_type = other RNA
aggaaaaagtacaggtgtga

SEQ ID NO: 5490 - RNA, 20 nt, synthetic construct
  source 1..20: mol_type = other RNA
ggaaaaagtacaggtgtgaa

SEQ ID NO: 5491 - RNA, 20 nt, synthetic construct
  source 1..20: mol_type = other RNA
aaagtacaggtgtgaagggc

SEQ ID NO: 5492 - RNA, 20 nt, synthetic construct
  source 1..20: mol_type = other RNA
atcccaatgcacagtgtatt

SEQ ID NO: 5493 - RNA, 20 nt, synthetic construct
  source 1..20: mol_type = other RNA
atacactgtgcattgggatt

SEQ ID NO: 5494 - RNA, 20 nt, synthetic construct
  source 1..20: mol_type = other RNA
ttccaaatacactgtgcatt

SEQ ID NO: 5495 - RNA, 20 nt, synthetic construct
  source 1..20: mol_type = other RNA
tttccaaatacactgtgcat

SEQ ID NO: 5496 - RNA, 20 nt, synthetic construct
  source 1..20: mol_type = other RNA
ccccttagcatacgccttgt

SEQ ID NO: 5497 - RNA, 20 nt, synthetic construct
  source 1..20: mol_type = other RNA
ccaacaaggcgtatgctaag

SEQ ID NO: 5498 - RNA, 20 nt, synthetic construct
  source 1..20: mol_type = other RNA
tccaacaaggcgtatgctaa

SEQ ID NO: 5499 - RNA, 20 nt, synthetic construct
  source 1..20: mol_type = other RNA
ttccaacaaggcgtatgcta

SEQ ID NO: 5500 - RNA, 20 nt, synthetic construct
  source 1..20: mol_type = other RNA
cttgttggaaatgtttgctt

SEQ ID NO: 5501 - RNA, 20 nt, synthetic construct
  source 1..20: mol_type = other RNA
caaagcaaacatttccaaca

SEQ ID NO: 5502 - RNA, 20 nt, synthetic construct
  source 1..20: mol_type = other RNA
gacattgagacagcattccc

SEQ ID NO: 5503 - RNA, 20 nt, synthetic construct
  source 1..20: mol_type = other RNA
gacagcattcccaggaacaa

SEQ ID NO: 5504 - RNA, 20 nt, synthetic construct
  source 1..20: mol_type = other RNA
gcattcccaggaacaaaggc

SEQ ID NO: 5505 - RNA, 20 nt, synthetic construct
  source 1..20: mol_type = other RNA
cattcccaggaacaaaggct

SEQ ID NO: 5506 - RNA, 20 nt, synthetic construct
  source 1..20: mol_type = other RNA
attcccaggaacaaaggctg

SEQ ID NO: 5507 - RNA, 20 nt, synthetic construct
  source 1..20: mol_type = other RNA
ttcccaggaacaaaggctgg

SEQ ID NO: 5508 - RNA, 20 nt, synthetic construct
  source 1..20: mol_type = other RNA
ccaggaacaaaggctggggg

SEQ ID NO: 5509 - RNA, 20 nt, synthetic construct
  source 1..20: mol_type = other RNA
ggaacaaaggctgggggtgg

SEQ ID NO: 5510 - RNA, 20 nt, synthetic construct
  source 1..20: mol_type = other RNA
cacccccagcctttgttcct

SEQ ID NO: 5511 - RNA, 20 nt, synthetic construct
  source 1..20: mol_type = other RNA
ccacccccagcctttgttcc

SEQ ID NO: 5512 - RNA, 20 nt, synthetic construct
  source 1..20: mol_type = other RNA
caaaggctgggggtggaggg

SEQ ID NO: 5513 - RNA, 20 nt, synthetic construct
  source 1..20: mol_type = other RNA
aggctgggggtggagggtgg

SEQ ID NO: 5514 - RNA, 20 nt, synthetic construct
  source 1..20: mol_type = other RNA
ctgggggtggagggtggagg

SEQ ID NO: 5515 - RNA, 20 nt, synthetic construct
  source 1..20: mol_type = other RNA
tgggggtggagggtggagga

SEQ ID NO: 5516 - RNA, 20 nt, synthetic construct
  source 1..20: mol_type = other RNA
tggagggtggaggagggagc

SEQ ID NO: 5517 - RNA, 20 nt, synthetic construct
  source 1..20: mol_type = other RNA
gagcaggaacagcccctgtc

SEQ ID NO: 5518 - RNA, 20 nt, synthetic construct
  source 1..20: mol_type = other RNA
cttgcagttcttccagacag

SEQ ID NO: 5519 - RNA, 20 nt, synthetic construct
  source 1..20: mol_type = other RNA
acttgcagttcttccagaca

SEQ ID NO: 5520 - RNA, 20 nt, synthetic construct
  source 1..20: mol_type = other RNA
aacttgcagttcttccagac

SEQ ID NO: 5521 - RNA, 20 nt, synthetic construct
  source 1..20: mol_type = other RNA
tggaagaactgcaagttctg

SEQ ID NO: 5522 - RNA, 20 nt, synthetic construct
  source 1..20: mol_type = other RNA
acaggacacatttcttgttc

SEQ ID NO: 5523 - RNA, 20 nt, synthetic construct
  source 1..20: mol_type = other RNA
gtgtcctgttcccgtgctcc

SEQ ID NO: 5524 - RNA, 20 nt, synthetic construct
  source 1..20: mol_type = other RNA
gcagccaggagcacgggaac

SEQ ID NO: 5525 - RNA, 20 nt, synthetic construct
  source 1..20: mol_type = other RNA
cccgtgctcctggctgcagc

SEQ ID NO: 5526 - RNA, 20 nt, synthetic construct
  source 1..20: mol_type = other RNA
ccgtgctcctggctgcagct

SEQ ID NO: 5527 - RNA, 20 nt, synthetic construct
  source 1..20: mol_type = other RNA
ccagctgcagccaggagcac

SEQ ID NO: 5528 - RNA, 20 nt, synthetic construct
  source 1..20: mol_type = other RNA
cccagctgcagccaggagca

SEQ ID NO: 5529 - RNA, 20 nt, synthetic construct
  source 1..20: mol_type = other RNA
gaagcttcccagctgcagcc

SEQ ID NO: 5530 - RNA, 20 nt, synthetic construct
  source 1..20: mol_type = other RNA
gctgggaagcttcttcagaa

SEQ ID NO: 5531 - RNA, 20 nt, synthetic construct
  source 1..20: mol_type = other RNA
tcttcagaaaggagacctcc

SEQ ID NO: 5532 - RNA, 20 nt, synthetic construct
  source 1..20: mol_type = other RNA
ggagacctcccggccctcac

SEQ ID NO: 5533 - RNA, 20 nt, synthetic construct
  source 1..20: mol_type = other RNA
gagacctcccggccctcacc

SEQ ID NO: 5534 - RNA, 20 nt, synthetic construct
  source 1..20: mol_type = other RNA
tcccggccctcaccgggatc

SEQ ID NO: 5535 - RNA, 20 nt, synthetic construct
  source 1..20: mol_type = other RNA
agatcccggtgagggccggg

SEQ ID NO: 5536 - RNA, 20 nt, synthetic construct
  source 1..20: mol_type = other RNA
gccagatcccggtgagggcc

SEQ ID NO: 5537 - RNA, 20 nt, synthetic construct
  source 1..20: mol_type = other RNA
agccagatcccggtgagggc

SEQ ID NO: 5538 - RNA, 20 nt, synthetic construct
  source 1..20: mol_type = other RNA
ggaaagccagatcccggtga

SEQ ID NO: 5539 - RNA, 20 nt, synthetic construct
  source 1..20: mol_type = other RNA
aggaaagccagatcccggtg

SEQ ID NO: 5540 - RNA, 20 nt, synthetic construct
  source 1..20: mol_type = other RNA
agggaaggaaagccagatcc

SEQ ID NO: 5541 - RNA, 20 nt, synthetic construct
  source 1..20: mol_type = other RNA
acagatgtggtgggaaggga

SEQ ID NO: 5542 - RNA, 20 nt, synthetic construct
  source 1..20: mol_type = other RNA
ataaacagatgtggtgggaa

SEQ ID NO: 5543 - RNA, 20 nt, synthetic construct
  source 1..20: mol_type = other RNA
tataaacagatgtggtggga

SEQ ID NO: 5544 - RNA, 20 nt, synthetic construct
  source 1..20: mol_type = other RNA
caccacatctgtttatacaa

SEQ ID NO: 5545 - RNA, 20 nt, synthetic construct
  source 1..20: mol_type = other RNA
cacatctgtttatacaaagg

SEQ ID NO: 5546 - RNA, 20 nt, synthetic construct
  source 1..20: mol_type = other RNA
ctttgtataaacagatgtgg

SEQ ID NO: 5547 - RNA, 20 nt, synthetic construct
  source 1..20: mol_type = other RNA
ctcctttgtataaacagatg

SEQ ID NO: 5548 - RNA, 20 nt, synthetic construct
  source 1..20: mol_type = other RNA
atacaaaggagggccgctga

SEQ ID NO: 5549 - RNA, 20 nt, synthetic construct
  source 1..20: mol_type = other RNA
cggttatgtttgtccttcag

SEQ ID NO: 5550 - RNA, 20 nt, synthetic construct
  source 1..20: mol_type = other RNA
gtttactgcgagtcccatgc

SEQ ID NO: 5551 - RNA, 20 nt, synthetic construct
  source 1..20: mol_type = other RNA
tttactgcgagtcccatgct

SEQ ID NO: 5552 - RNA, 20 nt, synthetic construct
  source 1..20: mol_type = other RNA
tgcgagtcccatgctgggcc

SEQ ID NO: 5553 - RNA, 20 nt, synthetic construct
  source 1..20: mol_type = other RNA
ctgagctccaggcccagcat

SEQ ID NO: 5554 - RNA, 20 nt, synthetic construct
  source 1..20: mol_type = other RNA
tctgagctccaggcccagca

SEQ ID NO: 5555 - RNA, 20 nt, synthetic construct
  source 1..20: mol_type = other RNA
caaatctgtatctgagctcc

SEQ ID NO: 5556 - RNA, 20 nt, synthetic construct
  source 1..20: mol_type = other RNA
atacagatttgccctcacca

SEQ ID NO: 5557 - RNA, 20 nt, synthetic construct
  source 1..20: mol_type = other RNA
cagatttgccctcaccatgg

SEQ ID NO: 5558 - RNA, 20 nt, synthetic construct
  source 1..20: mol_type = other RNA
atcttcagcctccatggtga

SEQ ID NO: 5559 - RNA, 20 nt, synthetic construct
  source 1..20: mol_type = other RNA
tatcttcagcctccatggtg

SEQ ID NO: 5560 - RNA, 20 nt, synthetic construct
  source 1..20: mol_type = other RNA
ctatttatcttcagcctcca

SEQ ID NO: 5561 - RNA, 20 nt, synthetic construct
  source 1..20: mol_type = other RNA
taaatagatgatcccagaaa

SEQ ID NO: 5562 - RNA, 20 nt, synthetic construct
  source 1..20: mol_type = other RNA
atgatcccagaaaaggaaag

SEQ ID NO: 5563 - RNA, 20 nt, synthetic construct
  source 1..20: mol_type = other RNA
tgatcccagaaaaggaaaga

SEQ ID NO: 5564 - RNA, 20 nt, synthetic construct
  source 1..20: mol_type = other RNA
cccagaaaaggaaagaggga

SEQ ID NO: 5565 - RNA, 20 nt, synthetic construct
  source 1..20: mol_type = other RNA
ccttccctctttccttttct

SEQ ID NO: 5566 - RNA, 20 nt, synthetic construct
  source 1..20: mol_type = other RNA
aaaggaaagagggaaggccc

SEQ ID NO: 5567 - RNA, 20 nt, synthetic construct
  source 1..20: mol_type = other RNA
aaggaaagagggaaggccct

SEQ ID NO: 5568 - RNA, 20 nt, synthetic construct
  source 1..20: mol_type = other RNA
aaagagggaaggccctggga

SEQ ID NO: 5569 - RNA, 20 nt, synthetic construct
  source 1..20: mol_type = other RNA
gccctgggatggtatagagc

SEQ ID NO: 5570 - RNA, 20 nt, synthetic construct
  source 1..20: mol_type = other RNA
ggatggtatagagctggttg

SEQ ID NO: 5571 - RNA, 20 nt, synthetic construct
  source 1..20: mol_type = other RNA
gatggtatagagctggttga

SEQ ID NO: 5572 - RNA, 20 nt, synthetic construct
  source 1..20: mol_type = other RNA
atggtatagagctggttgag

SEQ ID NO: 5573 - RNA, 20 nt, synthetic construct
  source 1..20: mol_type = other RNA
ttgaggggtttactcatgaa

SEQ ID NO: 5574 - RNA, 20 nt, synthetic construct
  source 1..20: mol_type = other RNA
cccaaaaagccatgtagtaa

SEQ ID NO: 5575 - RNA, 20 nt, synthetic construct
  source 1..20: mol_type = other RNA
ccaaaaagccatgtagtaac

SEQ ID NO: 5576 - RNA, 20 nt, synthetic construct
  source 1..20: mol_type = other RNA
ccgttactacatggcttttt

SEQ ID NO: 5577 - RNA, 20 nt, synthetic construct
  source 1..20: mol_type = other RNA
cccgttactacatggctttt

SEQ ID NO: 5578 - RNA, 20 nt, synthetic construct
  source 1..20: mol_type = other RNA
taaatctgcccgttactaca

SEQ ID NO: 5579 - RNA, 20 nt, synthetic construct
  source 1..20: mol_type = other RNA
ttacgtttgaatttaaactc

SEQ ID NO: 5580 - RNA, 20 nt, synthetic construct
  source 1..20: mol_type = other RNA
cactctcatatattaacaca

SEQ ID NO: 5581 - RNA, 20 nt, synthetic construct
  source 1..20: mol_type = other RNA
gtgcacctaaagcaattgca

SEQ ID NO: 5582 - RNA, 20 nt, synthetic construct
  source 1..20: mol_type = other RNA
cacctaaagcaattgcaagg

SEQ ID NO: 5583 - RNA, 20 nt, synthetic construct
  source 1..20: mol_type = other RNA
acctaaagcaattgcaaggc

SEQ ID NO: 5584 - RNA, 20 nt, synthetic construct
  source 1..20: mol_type = other RNA
acccgccttgcaattgcttt

SEQ ID NO: 5585 - RNA, 20 nt, synthetic construct
  source 1..20: mol_type = other RNA
gtatttaaaaatgtttcttt

SEQ ID NO: 5586 - RNA, 20 nt, synthetic construct
  source 1..20: mol_type = other RNA
aatagccatgattttctgtt

SEQ ID NO: 5587 - RNA, 20 nt, synthetic construct
  source 1..20: mol_type = other RNA
atagccatgattttctgttt

SEQ ID NO: 5588 - RNA, 20 nt, synthetic construct
  source 1..20: mol_type = other RNA
tagccatgattttctgtttg

SEQ ID NO: 5589 - RNA, 20 nt, synthetic construct
  source 1..20: mol_type = other RNA
aggccccaaacagaaaatca

SEQ ID NO: 5590 - RNA, 20 nt, synthetic construct
  source 1..20: mol_type = other RNA
tctgtttggggcctctaaca

SEQ ID NO: 5591 - RNA, 20 nt, synthetic construct
  source 1..20: mol_type = other RNA
ctgtttggggcctctaacat

SEQ ID NO: 5592 - RNA, 20 nt, synthetic construct
  source 1..20: mol_type = other RNA
tgtttggggcctctaacatg

SEQ ID NO: 5593 - RNA, 20 nt, synthetic construct
  source 1..20: mol_type = other RNA
gcctctaacatggggatagt

SEQ ID NO: 5594 - RNA, 20 nt, synthetic construct
  source 1..20: mol_type = other RNA
tccaactatccccatgttag

SEQ ID NO: 5595 - RNA, 20 nt, synthetic construct
  source 1..20: mol_type = other RNA
attacatgaaaacataacac

SEQ ID NO: 5596 - RNA, 20 nt, synthetic construct
  source 1..20: mol_type = other RNA
gttttcatgtaatagtgtct

SEQ ID NO: 5597 - RNA, 20 nt, synthetic construct
  source 1..20: mol_type = other RNA
taatagtgtcttggagaatg

SEQ ID NO: 5598 - RNA, 20 nt, synthetic construct
  source 1..20: mol_type = other RNA
ttggagaatgaggacttttg

SEQ ID NO: 5599 - RNA, 20 nt, synthetic construct
  source 1..20: mol_type = other RNA
aggatctgcaactactattt

SEQ ID NO: 5600 - RNA, 20 nt, synthetic construct
  source 1..20: mol_type = other RNA
caggatctgcaactactatt

SEQ ID NO: 5601 - RNA, 20 nt, synthetic construct
  source 1..20: mol_type = other RNA
tgttttttactaagctgtca

SEQ ID NO: 5602 - RNA, 20 nt, synthetic construct
  source 1..20: mol_type = other RNA
atgacagcttagtaaaaaac

SEQ ID NO: 5603 - RNA, 20 nt, synthetic construct
  source 1..20: mol_type = other RNA
tttacttgtaaaaactattt

SEQ ID NO: 5604 - RNA, 20 nt, synthetic construct
  source 1..20: mol_type = other RNA
acagttagtgagagccttta

SEQ ID NO: 5605 - RNA, 20 nt, synthetic construct
  source 1..20: mol_type = other RNA
cagttagtgagagcctttat

SEQ ID NO: 5606 - RNA, 20 nt, synthetic construct
  source 1..20: mol_type = other RNA
ataataaagatctcccataa

SEQ ID NO: 5607 - RNA, 20 nt, synthetic construct
  source 1..20: mol_type = other RNA
ggagatctttattatttatc

SEQ ID NO: 5608 - RNA, 20 nt, synthetic construct
  source 1..20: mol_type = other RNA
tcctattatcctccagcctc

SEQ ID NO: 5609 - RNA, 20 nt, synthetic construct
  source 1..20: mol_type = other RNA
cctattatcctccagcctct

SEQ ID NO: 5610 - RNA, 20 nt, synthetic construct
  source 1..20: mol_type = other RNA
cccagaggctggaggataat

SEQ ID NO: 5611 - RNA, 20 nt, synthetic construct
  source 1..20: mol_type = other RNA
tttgcatacccagaggctgg

SEQ ID NO: 5612 - RNA, 20 nt, synthetic construct
  source 1..20: mol_type = other RNA
tggtttgcatacccagaggc

SEQ ID NO: 5613 - RNA, 20 nt, synthetic construct
  source 1..20: mol_type = other RNA
gttttggtttgcatacccag

SEQ ID NO: 5614 - RNA, 20 nt, synthetic construct
  source 1..20: mol_type = other RNA
actagattaagtgcttgttt

SEQ ID NO: 5615 - RNA, 20 nt, synthetic construct
  source 1..20: mol_type = other RNA
ccttaatacaaagcaaaaaa

SEQ ID NO: 5616 - RNA, 20 nt, synthetic construct
  source 1..20: mol_type = other RNA
cttaatacaaagcaaaaaaa

SEQ ID NO: 5617 - RNA, 20 nt, synthetic construct
  source 1..20: mol_type = other RNA
cctttttttgctttgtatta

SEQ ID NO: 5618 - RNA, 20 nt, synthetic construct
  source 1..20: mol_type = other RNA
tacaaagcaaaaaaagggtt

SEQ ID NO: 5619 - RNA, 20 nt, synthetic construct
  source 1..20: mol_type = other RNA
aaaaaaagggtttggacttt

SEQ ID NO: 5620 - RNA, 20 nt, synthetic construct
  source 1..20: mol_type = other RNA
aaaaaagggtttggactttt

SEQ ID NO: 5621 - RNA, 20 nt, synthetic construct
  source 1..20: mol_type = other RNA
aaaaagggtttggacttttg

SEQ ID NO: 5622 - RNA, 20 nt, synthetic construct
  source 1..20: mol_type = other RNA
attagaatgtcagaactaaa

SEQ ID NO: 5623 - RNA, 20 nt, synthetic construct
  source 1..20: mol_type = other RNA
ttagaatgtcagaactaaaa

SEQ ID NO: 5624 - RNA, 20 nt, synthetic construct
  source 1..20: mol_type = other RNA
tataggatgagcaaaagcta

SEQ ID NO: 5625 - RNA, 20 nt, synthetic construct
  source 1..20: mol_type = other RNA
cctatagtgcttgtgacctg

SEQ ID NO: 5626 - RNA, 20 nt, synthetic construct
  source 1..20: mol_type = other RNA
ctatagtgcttgtgacctga

SEQ ID NO: 5627 - RNA, 20 nt, synthetic construct
  source 1..20: mol_type = other RNA
cctcaggtcacaagcactat

SEQ ID NO: 5628 - RNA, 20 nt, synthetic construct
  source 1..20: mol_type = other RNA
gagggtcttttctccccaca

SEQ ID NO: 5629 - RNA, 20 nt, synthetic construct
  source 1..20: mol_type = other RNA
tgtggggagaaaagaccctc

SEQ ID NO: 5630 - RNA, 20 nt, synthetic construct
  source 1..20: mol_type = other RNA
gtgttgcttgcatccatgtg

SEQ ID NO: 5631 - RNA, 20 nt, synthetic construct
  source 1..20: mol_type = other RNA
ggtgttgcttgcatccatgt

SEQ ID NO: 5632 - RNA, 20 nt, synthetic construct
  source 1..20: mol_type = other RNA
tggatgcaagcaacacccct

SEQ ID NO: 5633 - RNA, 20 nt, synthetic construct
  source 1..20: mol_type = other RNA
tggtttgattcagctcccag

SEQ ID NO: 5634 - RNA, 20 nt, synthetic construct
  source 1..20: mol_type = other RNA
gtggtttgattcagctccca

SEQ ID NO: 5635 - RNA, 20 nt, synthetic construct
  source 1..20: mol_type = other RNA
ggtggtttgattcagctccc

SEQ ID NO: 5636 - RNA, 20 nt, synthetic construct
  source 1..20: mol_type = other RNA
tgaatcaaaccacccagcta

SEQ ID NO: 5637 - RNA, 20 nt, synthetic construct
  source 1..20: mol_type = other RNA
gaatcaaaccacccagctaa

SEQ ID NO: 5638 - RNA, 20 nt, synthetic construct
  source 1..20: mol_type = other RNA
aatcaaaccacccagctaag

SEQ ID NO: 5639 - RNA, 20 nt, synthetic construct
  source 1..20: mol_type = other RNA
caaaccacccagctaagggg

SEQ ID NO: 5640 - RNA, 20 nt, synthetic construct
  source 1..20: mol_type = other RNA
aaaccacccagctaagggga

SEQ ID NO: 5641 - RNA, 20 nt, synthetic construct
  source 1..20: mol_type = other RNA
ccagctaaggggagggctgc

SEQ ID NO: 5642 - RNA, 20 nt, synthetic construct
  source 1..20: mol_type = other RNA
cagctaaggggagggctgct

SEQ ID NO: 5643 - RNA, 20 nt, synthetic construct
  source 1..20: mol_type = other RNA
agctaaggggagggctgctg

SEQ ID NO: 5644 - RNA, 20 nt, synthetic construct
  source 1..20: mol_type = other RNA
gctaaggggagggctgctgg

SEQ ID NO: 5645 - RNA, 20 nt, synthetic construct
  source 1..20: mol_type = other RNA
cagcagccctccccttagct

SEQ ID NO: 5646 - RNA, 20 nt, synthetic construct
  source 1..20: mol_type = other RNA
ccagcagccctccccttagc

SEQ ID NO: 5647 - RNA, 20 nt, synthetic construct
  source 1..20: mol_type = other RNA
gggggaagctgctaaatgag

SEQ ID NO: 5648 - RNA, 20 nt, synthetic construct
  source 1..20: mol_type = other RNA
gctaaatgagaggagctgct

SEQ ID NO: 5649 - RNA, 20 nt, synthetic construct
  source 1..20: mol_type = other RNA
agaggagctgcttggcttcc

SEQ ID NO: 5650 - RNA, 20 nt, synthetic construct
  source 1..20: mol_type = other RNA
gaggagctgcttggcttccc

SEQ ID NO: 5651 - RNA, 20 nt, synthetic construct
  source 1..20: mol_type = other RNA
gctgcttggcttcccgggtc

SEQ ID NO: 5652 - RNA, 20 nt, synthetic construct
  source 1..20: mol_type = other RNA
cttggcttcccgggtcaggt

SEQ ID NO: 5653 - RNA, 20 nt, synthetic construct
  source 1..20: mol_type = other RNA
gcttcccgggtcaggttggt

SEQ ID NO: 5654 - RNA, 20 nt, synthetic construct
  source 1..20: mol_type = other RNA
cccgggtcaggttggttggt

SEQ ID NO: 5655 - RNA, 20 nt, synthetic construct
  source 1..20: mol_type = other RNA
ccaaccaaccaacctgaccc

SEQ ID NO: 5656 - RNA, 20 nt, synthetic construct
  source 1..20: mol_type = other RNA
accaaccaaccaacctgacc

SEQ ID NO: 5657 - RNA, 20 nt, synthetic construct
  source 1..20: mol_type = other RNA
agactaaatgtaccaaagaa

SEQ ID NO: 5658 - RNA, 20 nt, synthetic construct
  source 1..20: mol_type = other RNA
gactaaatgtaccaaagaaa

SEQ ID NO: 5659 - RNA, 20 nt, synthetic construct
  source 1..20: mol_type = other RNA
catttgttagtccctttctt

SEQ ID NO: 5660 - RNA, 20 nt, synthetic construct
  source 1..20: mol_type = other RNA
caaatgaatcctgctcagtc

SEQ ID NO: 5661 - RNA, 20 nt, synthetic construct
  source 1..20: mol_type = other RNA
aaatgaatcctgctcagtct

SEQ ID NO: 5662 - RNA, 20 nt, synthetic construct
  source 1..20: mol_type = other RNA
aatgaatcctgctcagtctg

SEQ ID NO: 5663 - RNA, 20 nt, synthetic construct
  source 1..20: mol_type = other RNA
agtagggccccagactgagc

SEQ ID NO: 5664 - RNA, 20 nt, synthetic construct
  source 1..20: mol_type = other RNA
aggttggcagaatgtgagta

SEQ ID NO: 5665 - RNA, 20 nt, synthetic construct
  source 1..20: mol_type = other RNA
taggttggcagaatgtgagt

SEQ ID NO: 5666 - RNA, 20 nt, synthetic construct
  source 1..20: mol_type = other RNA
acattctgccaacctagtgc

SEQ ID NO: 5667 - RNA, 20 nt, synthetic construct
  source 1..20: mol_type = other RNA
ggaggcttccagcactaggt

SEQ ID NO: 5668 - RNA, 20 nt, synthetic construct
  source 1..20: mol_type = other RNA
tttaggaggcttccagcact

SEQ ID NO: 5669 - RNA, 20 nt, synthetic construct
  source 1..20: mol_type = other RNA
tgcttctggatttatttagg

SEQ ID NO: 5670 - RNA, 20 nt, synthetic construct
  source 1..20: mol_type = other RNA
gtttgcttctggatttattt

SEQ ID NO: 5671 - RNA, 20 nt, synthetic construct
  source 1..20: mol_type = other RNA
agatgctataggtttgcttc

SEQ ID NO: 5672 - RNA, 20 nt, synthetic construct
  source 1..20: mol_type = other RNA
agggagatcttagatgctat

SEQ ID NO: 5673 - RNA, 20 nt, synthetic construct
  source 1..20: mol_type = other RNA
tctatcaaatcatatctgaa

SEQ ID NO: 5674 - RNA, 20 nt, synthetic construct
  source 1..20: mol_type = other RNA
ttctatcaaatcatatctga

SEQ ID NO: 5675 - RNA, 20 nt, synthetic construct
  source 1..20: mol_type = other RNA
gatagaagagaagccttgca

SEQ ID NO: 5676 - RNA, 20 nt, synthetic construct
  source 1..20: mol_type = other RNA
gcatgaattaaagccatgca

SEQ ID NO: 5677 - RNA, 20 nt, synthetic construct
  source 1..20: mol_type = other RNA
gcagctgcgtcttcaggata

SEQ ID NO: 5678 - RNA, 20 nt, synthetic construct
  source 1..20: mol_type = other RNA
aagacgcagctgcaactcag

SEQ ID NO: 5679 - RNA, 20 nt, synthetic construct
  source 1..20: mol_type = other RNA
tgagttgcagctgcgtcttc

SEQ ID NO: 5680 - RNA, 20 nt, synthetic construct
  source 1..20: mol_type = other RNA
aggtcatttttgtaaccaag

SEQ ID NO: 5681 - RNA, 20 nt, synthetic construct
  source 1..20: mol_type = other RNA
ggtcatttttgtaaccaagt

SEQ ID NO: 5682 - RNA, 20 nt, synthetic construct
  source 1..20: mol_type = other RNA
gagagaaaaaaaatcccact

SEQ ID NO: 5683 - RNA, 20 nt, synthetic construct
  source 1..20: mol_type = other RNA
tatttttctaggggaatggt

SEQ ID NO: 5684 - RNA, 20 nt, synthetic construct
  source 1..20: mol_type = other RNA
atatttttctaggggaatgg

SEQ ID NO: 5685 - RNA, 20 nt, synthetic construct
  source 1..20: mol_type = other RNA
ttcccctagaaaaatatgtc

SEQ ID NO: 5686 - RNA, 20 nt, synthetic construct
  source 1..20: mol_type = other RNA
gacatatttttctaggggaa

SEQ ID NO: 5687 - RNA, 20 nt, synthetic construct
  source 1..20: mol_type = other RNA
ggccagacatatttttctag

SEQ ID NO: 5688 - RNA, 20 nt, synthetic construct
  source 1..20: mol_type = other RNA
tggccagacatatttttcta

SEQ ID NO: 5689 - RNA, 20 nt, synthetic construct
  source 1..20: mol_type = other RNA
ttggccagacatatttttct

SEQ ID NO: 5690 - RNA, 20 nt, synthetic construct
  source 1..20: mol_type = other RNA
aaatatgtctggccaaaagc

SEQ ID NO: 5691 - RNA, 20 nt, synthetic construct
  source 1..20: mol_type = other RNA
tggccaaaagctggctctgc

SEQ ID NO: 5692 - RNA, 20 nt, synthetic construct
  source 1..20: mol_type = other RNA
ccaaaagctggctctgcagg

SEQ ID NO: 5693 - RNA, 20 nt, synthetic construct
  source 1..20: mol_type = other RNA
ccacctgcagagccagcttt

SEQ ID NO: 5694 - RNA, 20 nt, synthetic construct
  source 1..20: mol_type = other RNA
ggctctgcaggtggtactgc

SEQ ID NO: 5695 - RNA, 20 nt, synthetic construct
  source 1..20: mol_type = other RNA
ctgcaggtggtactgctgga

SEQ ID NO: 5696 - RNA, 20 nt, synthetic construct
  source 1..20: mol_type = other RNA
tggtactgctggaaggtgat

SEQ ID NO: 5697 - RNA, 20 nt, synthetic construct
  source 1..20: mol_type = other RNA
aggagatgctgtaggggctg

SEQ ID NO: 5698 - RNA, 20 nt, synthetic construct
  source 1..20: mol_type = other RNA
agctggaggagatgctgtag

SEQ ID NO: 5699 - RNA, 20 nt, synthetic construct
  source 1..20: mol_type = other RNA
aagctggaggagatgctgta

SEQ ID NO: 5700 - RNA, 20 nt, synthetic construct
  source 1..20: mol_type = other RNA
aaagctggaggagatgctgt

SEQ ID NO: 5701 - RNA, 20 nt, synthetic construct
  source 1..20: mol_type = other RNA
ctcctccagctttgtcccta

SEQ ID NO: 5702 - RNA, 20 nt, synthetic construct
  source 1..20: mol_type = other RNA
gtccttagggacaaagctgg

SEQ ID NO: 5703 - RNA, 20 nt, synthetic construct
  source 1..20: mol_type = other RNA
agtgtccttagggacaaagc

SEQ ID NO: 5704 - RNA, 20 nt, synthetic construct
  source 1..20: mol_type = other RNA
aggagagagtagtgtcctta

SEQ ID NO: 5705 - RNA, 20 nt, synthetic construct
  source 1..20: mol_type = other RNA
caggagagagtagtgtcctt

SEQ ID NO: 5706 - RNA, 20 nt, synthetic construct
  source 1..20: mol_type = other RNA
gtctgcagctttgctggaac

SEQ ID NO: 5707 - RNA, 20 nt, synthetic construct
  source 1..20: mol_type = other RNA
tcatgcgtctgcagctttgc

SEQ ID NO: 5708 - RNA, 20 nt, synthetic construct
  source 1..20: mol_type = other RNA
ccatctgcttctccttccag

SEQ ID NO: 5709 - RNA, 20 nt, synthetic construct
  source 1..20: mol_type = other RNA
cctctggaaggagaagcaga

SEQ ID NO: 5710 - RNA, 20 nt, synthetic construct
  source 1..20: mol_type = other RNA
ttctccttccagaggcttct

SEQ ID NO: 5711 - RNA, 20 nt, synthetic construct
  source 1..20: mol_type = other RNA
tctccttccagaggcttctt

SEQ ID NO: 5712 - RNA, 20 nt, synthetic construct
  source 1..20: mol_type = other RNA
acacccaagaagcctctgga

SEQ ID NO: 5713 - RNA, 20 nt, synthetic construct
  source 1..20: mol_type = other RNA
acaaacacccaagaagcctc

SEQ ID NO: 5714 - RNA, 20 nt, synthetic construct
  source 1..20: mol_type = other RNA
gggtgtttgtaactgtatcc

SEQ ID NO: 5715 - RNA, 20 nt, synthetic construct
  source 1..20: mol_type = other RNA
ggtgtttgtaactgtatcca

SEQ ID NO: 5716 - RNA, 20 nt, synthetic construct
  source 1..20: mol_type = other RNA
taactgtatccagggattgc

SEQ ID NO: 5717 - RNA, 20 nt, synthetic construct
  source 1..20: mol_type = other RNA
gattgcaggataaaccttct

SEQ ID NO: 5718 - RNA, 20 nt, synthetic construct
  source 1..20: mol_type = other RNA
ttgcaaggagaaagcctaga

SEQ ID NO: 5719 - RNA, 20 nt, synthetic construct
  source 1..20: mol_type = other RNA
atattagcatgtaatttgca

SEQ ID NO: 5720 - RNA, 20 nt, synthetic construct
  source 1..20: mol_type = other RNA
atgctaatatgttgaacccc

SEQ ID NO: 5721 - RNA, 20 nt, synthetic construct
  source 1..20: mol_type = other RNA
ctaaaatctacgctgtcctg

SEQ ID NO: 5722 - RNA, 20 nt, synthetic construct
  source 1..20: mol_type = other RNA
tctaaaatctacgctgtcct

SEQ ID NO: 5723 - RNA, 20 nt, synthetic construct
  source 1..20: mol_type = other RNA
atctaaaatctacgctgtcc

SEQ ID NO: 5724 - RNA, 20 nt, synthetic construct
  source 1..20: mol_type = other RNA
cgtagattttagatccaccc

SEQ ID NO: 5725 - RNA, 20 nt, synthetic construct
  source 1..20: mol_type = other RNA
ccaggagttcttgtgtcttc

SEQ ID NO: 5726 - RNA, 20 nt, synthetic construct
  source 1..20: mol_type = other RNA
aagacacaagaactcctggg

SEQ ID NO: 5727 - RNA, 20 nt, synthetic construct
  source 1..20: mol_type = other RNA
ctgaagacacaagaactcct

SEQ ID NO: 5728 - RNA, 20 nt, synthetic construct
  source 1..20: mol_type = other RNA
cctgaagacacaagaactcc

SEQ ID NO: 5729 - RNA, 20 nt, synthetic construct
  source 1..20: mol_type = other RNA
gcctttccctctctctccac

SEQ ID NO: 5730 - RNA, 20 nt, synthetic construct
  source 1..20: mol_type = other RNA
acctgtggagagagagggaa

SEQ ID NO: 5731 - RNA, 20 nt, synthetic construct
  source 1..20: mol_type = other RNA
gagatacctgtggagagaga

SEQ ID NO: 5732 - RNA, 20 nt, synthetic construct
  source 1..20: mol_type = other RNA
agagatacctgtggagagag

SEQ ID NO: 5733 - RNA, 20 nt, synthetic construct
  source 1..20: mol_type = other RNA
tctccacaggtatctctgag

SEQ ID NO: 5734 - RNA, 20 nt, synthetic construct
  source 1..20: mol_type = other RNA
gaaccactcagagatacctg

SEQ ID NO: 5735 - RNA, 20 nt, synthetic construct
  source 1..20: mol_type = other RNA
tctctgagtggttctaacct

SEQ ID NO: 5736 - RNA, 20 nt, synthetic construct
  source 1..20: mol_type = other RNA
tggttctaacctaggattcg

SEQ ID NO: 5737 - RNA, 20 nt, synthetic construct
  source 1..20: mol_type = other RNA
agaaaggcacctcgaatcct

SEQ ID NO: 5738 - RNA, 20 nt, synthetic construct
  source 1..20: mol_type = other RNA
atgaaaaaatacagaaagaa

SEQ ID NO: 5739 - RNA, 20 nt, synthetic construct
  source 1..20: mol_type = other RNA
gtattttttcatcattcacc

SEQ ID NO: 5740 - RNA, 20 nt, synthetic construct
  source 1..20: mol_type = other RNA
ttcaccaggtcccgagcaga

SEQ ID NO: 5741 - RNA, 20 nt, synthetic construct
  source 1..20: mol_type = other RNA
caggtcccgagcagatggtg

SEQ ID NO: 5742 - RNA, 20 nt, synthetic construct
  source 1..20: mol_type = other RNA
cacaccatctgctcgggacc

SEQ ID NO: 5743 - RNA, 20 nt, synthetic construct
  source 1..20: mol_type = other RNA
cacagccacaccatctgctc

SEQ ID NO: 5744 - RNA, 20 nt, synthetic construct
  source 1..20: mol_type = other RNA
gcacagccacaccatctgct

SEQ ID NO: 5745 - RNA, 20 nt, synthetic construct
  source 1..20: mol_type = other RNA
tcactcctcctatgtttcca

SEQ ID NO: 5746 - RNA, 20 nt, synthetic construct
  source 1..20: mol_type = other RNA
cctatgtttccatggaaaca

SEQ ID NO: 5747 - RNA, 20 nt, synthetic construct
  source 1..20: mol_type = other RNA
ctatgtttccatggaaacat

SEQ ID NO: 5748 - RNA, 20 nt, synthetic construct
  source 1..20: mol_type = other RNA
tgtttccatggaaacatagg

SEQ ID NO: 5749 - RNA, 20 nt, synthetic construct
  source 1..20: mol_type = other RNA
ccatgtttccatggaaacat

SEQ ID NO: 5750 - RNA, 20 nt, synthetic construct
  source 1..20: mol_type = other RNA
tccatggaaacatggggcat

SEQ ID NO: 5751 - RNA, 20 nt, synthetic construct
  source 1..20: mol_type = other RNA
ccatggaaacatggggcata

SEQ ID NO: 5752 - RNA, 20 nt, synthetic construct
  source 1..20: mol_type = other RNA
ccctatgccccatgtttcca

SEQ ID NO: 5753 - RNA, 20 nt, synthetic construct
  source 1..20: mol_type = other RNA
catagggaccatctccgcct

SEQ ID NO: 5754 - RNA, 20 nt, synthetic construct
  source 1..20: mol_type = other RNA
atagggaccatctccgcctt

SEQ ID NO: 5755 - RNA, 20 nt, synthetic construct
  source 1..20: mol_type = other RNA
cagagagcccaaggcggaga

SEQ ID NO: 5756 - RNA, 20 nt, synthetic construct
  source 1..20: mol_type = other RNA
tactgtcagagagcccaagg

SEQ ID NO: 5757 - RNA, 20 nt, synthetic construct
  source 1..20: mol_type = other RNA
ggctctctgacagtatcctc

SEQ ID NO: 5758 - RNA, 20 nt, synthetic construct
  source 1..20: mol_type = other RNA
gtactgaagttcttcgccag

SEQ ID NO: 5759 - RNA, 20 nt, synthetic construct
  source 1..20: mol_type = other RNA
agtggacaggctggggggag

SEQ ID NO: 5760 - RNA, 20 nt, synthetic construct
  source 1..20: mol_type = other RNA
cagtggacaggctgggggga

SEQ ID NO: 5761 - RNA, 20 nt, synthetic construct
  source 1..20: mol_type = other RNA
acagtggacaggctgggggg

SEQ ID NO: 5762 - RNA, 20 nt, synthetic construct
  source 1..20: mol_type = other RNA
cccagcctgtccactgtcct

SEQ ID NO: 5763 - RNA, 20 nt, synthetic construct
  source 1..20: mol_type = other RNA
ccagcctgtccactgtccta

SEQ ID NO: 5764 - RNA, 20 nt, synthetic construct
  source 1..20: mol_type = other RNA
aggacagtggacaggctggg

SEQ ID NO: 5765 - RNA, 20 nt, synthetic construct
  source 1..20: mol_type = other RNA
taggacagtggacaggctgg

SEQ ID NO: 5766 - RNA, 20 nt, synthetic construct
  source 1..20: mol_type = other RNA
ctaggacagtggacaggctg

SEQ ID NO: 5767 - RNA, 20 nt, synthetic construct
  source 1..20: mol_type = other RNA
cctaggacagtggacaggct

SEQ ID NO: 5768 - RNA, 20 nt, synthetic construct
  source 1..20: mol_type = other RNA
ccctaggacagtggacaggc

SEQ ID NO: 5769 - RNA, 20 nt, synthetic construct
  source 1..20: mol_type = other RNA
tgtccactgtcctagggagt

SEQ ID NO: 5770 - RNA, 20 nt, synthetic construct
  source 1..20: mol_type = other RNA
aactccctaggacagtggac

SEQ ID NO: 5771 - RNA, 20 nt, synthetic construct
  source 1..20: mol_type = other RNA
tctccaactccctaggacag

SEQ ID NO: 5772 - RNA, 20 nt, synthetic construct
  source 1..20: mol_type = other RNA
tagggagttggagacctttc

SEQ ID NO: 5773 - RNA, 20 nt, synthetic construct
  source 1..20: mol_type = other RNA
agggagttggagacctttct

SEQ ID NO: 5774 - RNA, 20 nt, synthetic construct
  source 1..20: mol_type = other RNA
gggagttggagacctttctg

SEQ ID NO: 5775 - RNA, 20 nt, synthetic construct
  source 1..20: mol_type = other RNA
agaaaggtctccaactccct

SEQ ID NO: 5776 - RNA, 20 nt, synthetic construct
  source 1..20: mol_type = other RNA
tttctggggccctagaagcc

SEQ ID NO: 5777 - RNA, 20 nt, synthetic construct
  source 1..20: mol_type = other RNA
ttctggggccctagaagcca

SEQ ID NO: 5778 - RNA, 20 nt, synthetic construct
  source 1..20: mol_type = other RNA
tggcttctagggccccagaa

SEQ ID NO: 5779 - RNA, 20 nt, synthetic construct
  source 1..20: mol_type = other RNA
tgaaatgaccctggcttcta

SEQ ID NO: 5780 - RNA, 20 nt, synthetic construct
  source 1..20: mol_type = other RNA
ctgaaatgaccctggcttct

SEQ ID NO: 5781 - RNA, 20 nt, synthetic construct
  source 1..20: mol_type = other RNA
gatgatctctgaaatgaccc

SEQ ID NO: 5782 - RNA, 20 nt, synthetic construct
  source 1..20: mol_type = other RNA
aaggacatactccctgcaaa

SEQ ID NO: 5783 - RNA, 20 nt, synthetic construct
  source 1..20: mol_type = other RNA
ccctgcaaatggttttgaac

SEQ ID NO: 5784 - RNA, 20 nt, synthetic construct
  source 1..20: mol_type = other RNA
gcaaatggttttgaactggc

SEQ ID NO: 5785 - RNA, 20 nt, synthetic construct
  source 1..20: mol_type = other RNA
caaatggttttgaactggct

SEQ ID NO: 5786 - RNA, 20 nt, synthetic construct
  source 1..20: mol_type = other RNA
gccagttcaaaaccatttgc

SEQ ID NO: 5787 - RNA, 20 nt, synthetic construct
  source 1..20: mol_type = other RNA
gttttgaactggctgggaaa

SEQ ID NO: 5788 - RNA, 20 nt, synthetic construct
  source 1..20: mol_type = other RNA
ttgaactggctgggaaaagg

SEQ ID NO: 5789 - RNA, 20 nt, synthetic construct
  source 1..20: mol_type = other RNA
tgaactggctgggaaaagga

SEQ ID NO: 5790 - RNA, 20 nt, synthetic construct
  source 1..20: mol_type = other RNA
actggctgggaaaaggaggg

SEQ ID NO: 5791 - RNA, 20 nt, synthetic construct
  source 1..20: mol_type = other RNA
ctggctgggaaaaggaggga

SEQ ID NO: 5792 - RNA, 20 nt, synthetic construct
  source 1..20: mol_type = other RNA
gaaaaggagggagggtagaa

SEQ ID NO: 5793 - RNA, 20 nt, synthetic construct
  source 1..20: mol_type = other RNA
aaaaggagggagggtagaaa

SEQ ID NO: 5794 - RNA, 20 nt, synthetic construct
  source 1..20: mol_type = other RNA
aaaggagggagggtagaaag

SEQ ID NO: 5795 - RNA, 20 nt, synthetic construct
  source 1..20: mol_type = other RNA
aaggagggagggtagaaagg

SEQ ID NO: 5796 - RNA, 20 nt, synthetic construct
  source 1..20: mol_type = other RNA
tagaaagggggccaataccc

SEQ ID NO: 5797 - RNA, 20 nt, synthetic construct
  source 1..20: mol_type = other RNA
gggggccaataccccggtcg

SEQ ID NO: 5798 - RNA, 20 nt, synthetic construct
  source 1..20: mol_type = other RNA
ggggccaataccccggtcga

SEQ ID NO: 5799 - RNA, 20 nt, synthetic construct
  source 1..20: mol_type = other RNA
tcagccctcgaccggggtat

SEQ ID NO: 5800 - RNA, 20 nt, synthetic construct
  source 1..20: mol_type = other RNA
cagttctcagccctcgaccg

SEQ ID NO: 5801 - RNA, 20 nt, synthetic construct
  source 1..20: mol_type = other RNA
acagttctcagccctcgacc

SEQ ID NO: 5802 - RNA, 20 nt, synthetic construct
  source 1..20: mol_type = other RNA
aacagttctcagccctcgac

SEQ ID NO: 5803 - RNA, 20 nt, synthetic construct
  source 1..20: mol_type = other RNA
gggctgagaactgttttaga

SEQ ID NO: 5804 - RNA, 20 nt, synthetic construct
  source 1..20: mol_type = other RNA
gttttagaaggcaacatatt

SEQ ID NO: 5805 - RNA, 20 nt, synthetic construct
  source 1..20: mol_type = other RNA
tattatggaagctggctgca

SEQ ID NO: 5806 - RNA, 20 nt, synthetic construct
  source 1..20: mol_type = other RNA
ctattatggaagctggctgc

SEQ ID NO: 5807 - RNA, 20 nt, synthetic construct
  source 1..20: mol_type = other RNA
taatcagctattatggaagc

SEQ ID NO: 5808 - RNA, 20 nt, synthetic construct
  source 1..20: mol_type = other RNA
tgggcaataatcagctatta

SEQ ID NO: 5809 - RNA, 20 nt, synthetic construct
  source 1..20: mol_type = other RNA
gagcagctcttttgacatct

SEQ ID NO: 5810 - RNA, 20 nt, synthetic construct
  source 1..20: mol_type = other RNA
ggagcagctcttttgacatc

SEQ ID NO: 5811 - RNA, 20 nt, synthetic construct
  source 1..20: mol_type = other RNA
tgatgagcagactgaaccct

SEQ ID NO: 5812 - RNA, 20 nt, synthetic construct
  source 1..20: mol_type = other RNA
ttgaatgtaagtagttgctg

SEQ ID NO: 5813 - RNA, 20 nt, synthetic construct
  source 1..20: mol_type = other RNA
ttcactgacattctacaccc

SEQ ID NO: 5814 - RNA, 20 nt, synthetic construct
  source 1..20: mol_type = other RNA
tcactgacattctacaccct

SEQ ID NO: 5815 - RNA, 20 nt, synthetic construct
  source 1..20: mol_type = other RNA
accctgggaatgagtgtttc

SEQ ID NO: 5816 - RNA, 20 nt, synthetic construct
  source 1..20: mol_type = other RNA
ccctgggaatgagtgtttct

SEQ ID NO: 5817 - RNA, 20 nt, synthetic construct
  source 1..20: mol_type = other RNA
cccagaaacactcattccca

SEQ ID NO: 5818 - RNA, 20 nt, synthetic construct
  source 1..20: mol_type = other RNA
tcccagaaacactcattccc

SEQ ID NO: 5819 - RNA, 20 nt, synthetic construct
  source 1..20: mol_type = other RNA
aaaaaaaaaaaaaaaaaaaa

SEQ ID NO: 5820 - RNA, 20 nt, synthetic construct
  source 1..20: mol_type = other RNA
tttttttttttaacaaaacc

SEQ ID NO: 5821 - RNA, 20 nt, synthetic construct
  source 1..20: mol_type = other RNA
caaaaccaggtttttcccta

SEQ ID NO: 5822 - RNA, 20 nt, synthetic construct
  source 1..20: mol_type = other RNA
gcattccttagggaaaaacc

SEQ ID NO: 5823 - RNA, 20 nt, synthetic construct
  source 1..20: mol_type = other RNA
tggggaaggtgcattcctta

SEQ ID NO: 5824 - RNA, 20 nt, synthetic construct
  source 1..20: mol_type = other RNA
ttggggaaggtgcattcctt

SEQ ID NO: 5825 - RNA, 20 nt, synthetic construct
  source 1..20: mol_type = other RNA
gatgcgggaaactttgggga

SEQ ID NO: 5826 - RNA, 20 nt, synthetic construct
  source 1..20: mol_type = other RNA
ggaggatgcgggaaactttg

SEQ ID NO: 5827 - RNA, 20 nt, synthetic construct
  source 1..20: mol_type = other RNA
aggaggatgcgggaaacttt

SEQ ID NO: 5828 - RNA, 20 nt, synthetic construct
  source 1..20: mol_type = other RNA
caggaggatgcgggaaactt

SEQ ID NO: 5829 - RNA, 20 nt, synthetic construct
  source 1..20: mol_type = other RNA
ttatgtaggcaggaggatgc

SEQ ID NO: 5830 - RNA, 20 nt, synthetic construct
  source 1..20: mol_type = other RNA
attatgtaggcaggaggatg

SEQ ID NO: 5831 - RNA, 20 nt, synthetic construct
  source 1..20: mol_type = other RNA
aagtgaattatgtaggcagg

SEQ ID NO: 5832 - RNA, 20 nt, synthetic construct
  source 1..20: mol_type = other RNA
tataagtgaattatgtaggc

SEQ ID NO: 5833 - RNA, 20 nt, synthetic construct
  source 1..20: mol_type = other RNA
actatataagtgaattatgt

SEQ ID NO: 5834 - RNA, 20 nt, synthetic construct
  source 1..20: mol_type = other RNA
taattagattcagaagtctg

SEQ ID NO: 5835 - RNA, 20 nt, synthetic construct
  source 1..20: mol_type = other RNA
tctgtggaaacagcagagct

SEQ ID NO: 5836 - RNA, 20 nt, synthetic construct
  source 1..20: mol_type = other RNA
tggaaacagcagagctcggc

SEQ ID NO: 5837 - RNA, 20 nt, synthetic construct
  source 1..20: mol_type = other RNA
ggaaacagcagagctcggca

SEQ ID NO: 5838 - RNA, 20 nt, synthetic construct
  source 1..20: mol_type = other RNA
gcagagctcggcagggtcag

SEQ ID NO: 5839 - RNA, 20 nt, synthetic construct
  source 1..20: mol_type = other RNA
cagagctcggcagggtcaga

SEQ ID NO: 5840 - RNA, 20 nt, synthetic construct
  source 1..20: mol_type = other RNA
ggcagggtcagagggcaagc

SEQ ID NO: 5841 - RNA, 20 nt, synthetic construct
  source 1..20: mol_type = other RNA
gcagggtcagagggcaagca

SEQ ID NO: 5842 - RNA, 20 nt, synthetic construct
  source 1..20: mol_type = other RNA
aagcagggcagagaaaagag

SEQ ID NO: 5843 - RNA, 20 nt, synthetic construct
  source 1..20: mol_type = other RNA
agcagggcagagaaaagaga

SEQ ID NO: 5844 - RNA, 20 nt, synthetic construct
  source 1..20: mol_type = other RNA
gcagggcagagaaaagagag

SEQ ID NO: 5845 - RNA, 20 nt, synthetic construct
  source 1..20: mol_type = other RNA
agagaggggaaaatgagctc

SEQ ID NO: 5846 - RNA, 20 nt, synthetic construct
  source 1..20: mol_type = other RNA
gagaggggaaaatgagctcc

SEQ ID NO: 5847 - RNA, 20 nt, synthetic construct
  source 1..20: mol_type = other RNA
gggaaaatgagctccgggag

SEQ ID NO: 5848 - RNA, 20 nt, synthetic construct
  source 1..20: mol_type = other RNA
ggaaaatgagctccgggaga

SEQ ID NO: 5849 - RNA, 20 nt, synthetic construct
  source 1..20: mol_type = other RNA
gaaaatgagctccgggagag

SEQ ID NO: 5850 - RNA, 20 nt, synthetic construct
  source 1..20: mol_type = other RNA
atgagctccgggagagggga

SEQ ID NO: 5851 - RNA, 20 nt, synthetic construct
  source 1..20: mol_type = other RNA
tccgggagaggggaaggaag

SEQ ID NO: 5852 - RNA, 20 nt, synthetic construct
  source 1..20: mol_type = other RNA
gggagaggggaaggaagtgg

SEQ ID NO: 5853 - RNA, 20 nt, synthetic construct
  source 1..20: mol_type = other RNA
ggagaggggaaggaagtgga

SEQ ID NO: 5854 - RNA, 20 nt, synthetic construct
  source 1..20: mol_type = other RNA
tccacttccttcccctctcc

SEQ ID NO: 5855 - RNA, 20 nt, synthetic construct
  source 1..20: mol_type = other RNA
tgttttgtttggtacttgaa

SEQ ID NO: 5856 - RNA, 20 nt, synthetic construct
  source 1..20: mol_type = other RNA
ttgttttgtttggtacttga

SEQ ID NO: 5857 - RNA, 20 nt, synthetic construct
  source 1..20: mol_type = other RNA
gaaattatctttgttttgtt

SEQ ID NO: 5858 - RNA, 20 nt, synthetic construct
  source 1..20: mol_type = other RNA
aacaaagataatttcaaaag

SEQ ID NO: 5859 - RNA, 20 nt, synthetic construct
  source 1..20: mol_type = other RNA
ttctctaagcagtgttatag

SEQ ID NO: 5860 - RNA, 20 nt, synthetic construct
  source 1..20: mol_type = other RNA
aagagtgctttaaaataaag

SEQ ID NO: 5861 - RNA, 20 nt, synthetic construct
  source 1..20: mol_type = other RNA
gtgctttaaaataaagtgga

SEQ ID NO: 5862 - RNA, 20 nt, synthetic construct
  source 1..20: mol_type = other RNA
tgctttaaaataaagtggat

SEQ ID NO: 5863 - RNA, 20 nt, synthetic construct
  source 1..20: mol_type = other RNA
gctttaaaataaagtggatg

SEQ ID NO: 5864 - RNA, 20 nt, synthetic construct
  source 1..20: mol_type = other RNA
gggcataagcatgtatgtct

SEQ ID NO: 5865 - RNA, 20 nt, synthetic construct
  source 1..20: mol_type = other RNA
ttagttgctccttatacagc

SEQ ID NO: 5866 - RNA, 20 nt, synthetic construct
  source 1..20: mol_type = other RNA
ccttatacagccggtactaa

SEQ ID NO: 5867 - RNA, 20 nt, synthetic construct
  source 1..20: mol_type = other RNA
atacagccggtactaaaggc

SEQ ID NO: 5868 - RNA, 20 nt, synthetic construct
  source 1..20: mol_type = other RNA
cctttagtaccggctgtata

SEQ ID NO: 5869 - RNA, 20 nt, synthetic construct
  source 1..20: mol_type = other RNA
cagccggtactaaaggctgg

SEQ ID NO: 5870 - RNA, 20 nt, synthetic construct
  source 1..20: mol_type = other RNA
agccggtactaaaggctggt

SEQ ID NO: 5871 - RNA, 20 nt, synthetic construct
  source 1..20: mol_type = other RNA
cacccaccagcctttagtac

SEQ ID NO: 5872 - RNA, 20 nt, synthetic construct
  source 1..20: mol_type = other RNA
accacattttaaaaagaaaa

SEQ ID NO: 5873 - RNA, 20 nt, synthetic construct
  source 1..20: mol_type = other RNA
cattttaaaaagaaaaaggc

SEQ ID NO: 5874 - RNA, 20 nt, synthetic construct
  source 1..20: mol_type = other RNA
gcctttttctttttaaaatg

SEQ ID NO: 5875 - RNA, 20 nt, synthetic construct
  source 1..20: mol_type = other RNA
catactaaagttgaaaatgc

SEQ ID NO: 5876 - RNA, 20 nt, synthetic construct
  source 1..20: mol_type = other RNA
ctaaagttgaaaatgcaggc

SEQ ID NO: 5877 - RNA, 20 nt, synthetic construct
  source 1..20: mol_type = other RNA
agttgaaaatgcaggcagga

SEQ ID NO: 5878 - RNA, 20 nt, synthetic construct
  source 1..20: mol_type = other RNA
acatttacttttcataaaag

SEQ ID NO: 5879 - RNA, 20 nt, synthetic construct
  source 1..20: mol_type = other RNA
taaaatacatgatctgtgat

SEQ ID NO: 5880 - RNA, 20 nt, synthetic construct
  source 1..20: mol_type = other RNA
tatgccatgctgaccaatgt

SEQ ID NO: 5881 - RNA, 20 nt, synthetic construct
  source 1..20: mol_type = other RNA
atgccatgctgaccaatgtt

SEQ ID NO: 5882 - RNA, 20 nt, synthetic construct
  source 1..20: mol_type = other RNA
tgccatgctgaccaatgttg

SEQ ID NO: 5883 - RNA, 20 nt, synthetic construct
  source 1..20: mol_type = other RNA
gccatgctgaccaatgttgg

SEQ ID NO: 5884 - RNA, 20 nt, synthetic construct
  source 1..20: mol_type = other RNA
tcccccaacattggtcagca

SEQ ID NO: 5885 - RNA, 20 nt, synthetic construct
  source 1..20: mol_type = other RNA
atgagattatcccccaacat

SEQ ID NO: 5886 - RNA, 20 nt, synthetic construct
  source 1..20: mol_type = other RNA
atgagaagatcctttgatgc

SEQ ID NO: 5887 - RNA, 20 nt, synthetic construct
  source 1..20: mol_type = other RNA
gttcttgttaccagcatcaa

SEQ ID NO: 5888 - RNA, 20 nt, synthetic construct
  source 1..20: mol_type = other RNA
aagatttaagtcaggatgat

SEQ ID NO: 5889 - RNA, 20 nt, synthetic construct
  source 1..20: mol_type = other RNA
gggatattaagatttaagtc

SEQ ID NO: 5890 - RNA, 20 nt, synthetic construct
  source 1..20: mol_type = other RNA
ttaaatcttaatatccccac

SEQ ID NO: 5891 - RNA, 20 nt, synthetic construct
  source 1..20: mol_type = other RNA
agcatgacaaagaacctgtg

SEQ ID NO: 5892 - RNA, 20 nt, synthetic construct
  source 1..20: mol_type = other RNA
aagcatgacaaagaacctgt

SEQ ID NO: 5893 - RNA, 20 nt, synthetic construct
  source 1..20: mol_type = other RNA
gaagcatgacaaagaacctg

SEQ ID NO: 5894 - RNA, 20 nt, synthetic construct
  source 1..20: mol_type = other RNA
tgcttcttcaagatgtgccc

SEQ ID NO: 5895 - RNA, 20 nt, synthetic construct
  source 1..20: mol_type = other RNA
ggccattcatgcaagtttca

SEQ ID NO: 5896 - RNA, 20 nt, synthetic construct
  source 1..20: mol_type = other RNA
gaaacttgcatgaatggcca

SEQ ID NO: 5897 - RNA, 20 nt, synthetic construct
  source 1..20: mol_type = other RNA
tgaaacttgcatgaatggcc

SEQ ID NO: 5898 - RNA, 20 nt, synthetic construct
  source 1..20: mol_type = other RNA
gtccttgaaacttgcatgaa

SEQ ID NO: 5899 - RNA, 20 nt, synthetic construct
  source 1..20: mol_type = other RNA
actctgaatctgttgagaat

SEQ ID NO: 5900 - RNA, 20 nt, synthetic construct
  source 1..20: mol_type = other RNA
atgtctatattactgtcaac

SEQ ID NO: 5901 - RNA, 20 nt, synthetic construct
  source 1..20: mol_type = other RNA
tgtctatattactgtcaact

SEQ ID NO: 5902 - RNA, 20 nt, synthetic construct
  source 1..20: mol_type = other RNA
gtgcttttgggaggactaaa

SEQ ID NO: 5903 - RNA, 20 nt, synthetic construct
  source 1..20: mol_type = other RNA
agtcctcccaaaagcacatg

SEQ ID NO: 5904 - RNA, 20 nt, synthetic construct
  source 1..20: mol_type = other RNA
atacctcatgtgcttttggg

SEQ ID NO: 5905 - RNA, 20 nt, synthetic construct
  source 1..20: mol_type = other RNA
aacatacctcatgtgctttt

SEQ ID NO: 5906 - RNA, 20 nt, synthetic construct
  source 1..20: mol_type = other RNA
caacatacctcatgtgcttt

SEQ ID NO: 5907 - RNA, 20 nt, synthetic construct
  source 1..20: mol_type = other RNA
tgccattgtttttattttgc

SEQ ID NO: 5908 - RNA, 20 nt, synthetic construct
  source 1..20: mol_type = other RNA
cacctgcaaaataaaaacaa

SEQ ID NO: 5909 - RNA, 20 nt, synthetic construct
  source 1..20: mol_type = other RNA
ttttgcaggtgagtatgcta

SEQ ID NO: 5910 - RNA, 20 nt, synthetic construct
  source 1..20: mol_type = other RNA
aggtgagtatgctaaggaac

SEQ ID NO: 5911 - RNA, 20 nt, synthetic construct
  source 1..20: mol_type = other RNA
aagtgtcacaaacccaagca

SEQ ID NO: 5912 - RNA, 20 nt, synthetic construct
  source 1..20: mol_type = other RNA
aaacccaagcatggcagatc

SEQ ID NO: 5913 - RNA, 20 nt, synthetic construct
  source 1..20: mol_type = other RNA
aagcatggcagatcaggaat

SEQ ID NO: 5914 - RNA, 20 nt, synthetic construct
  source 1..20: mol_type = other RNA
attcctgatctgccatgctt

SEQ ID NO: 5915 - RNA, 20 nt, synthetic construct
  source 1..20: mol_type = other RNA
aattcctgatctgccatgct

SEQ ID NO: 5916 - RNA, 20 nt, synthetic construct
  source 1..20: mol_type = other RNA
tggcagatcaggaattggta

SEQ ID NO: 5917 - RNA, 20 nt, synthetic construct
  source 1..20: mol_type = other RNA
aggaattggtatggtattac

SEQ ID NO: 5918 - RNA, 20 nt, synthetic construct
  source 1..20: mol_type = other RNA
aagttgtgggaggtggagta

SEQ ID NO: 5919 - RNA, 20 nt, synthetic construct
  source 1..20: mol_type = other RNA
aaggcaaaagttgtgggagg

SEQ ID NO: 5920 - RNA, 20 nt, synthetic construct
  source 1..20: mol_type = other RNA
attaaggcaaaagttgtggg

SEQ ID NO: 5921 - RNA, 20 nt, synthetic construct
  source 1..20: mol_type = other RNA
ataattaaggcaaaagttgt

SEQ ID NO: 5922 - RNA, 20 nt, synthetic construct
  source 1..20: mol_type = other RNA
gataattaaggcaaaagttg

SEQ ID NO: 5923 - RNA, 20 nt, synthetic construct
  source 1..20: mol_type = other RNA
gccttaattatctatagcat

SEQ ID NO: 5924 - RNA, 20 nt, synthetic construct
  source 1..20: mol_type = other RNA
gccaatgctatagataatta

SEQ ID NO: 5925 - RNA, 20 nt, synthetic construct
  source 1..20: mol_type = other RNA
tggcgcattctcatgctcac

SEQ ID NO: 5926 - RNA, 20 nt, synthetic construct
  source 1..20: mol_type = other RNA
gaaagtaatacagtcccagt

SEQ ID NO: 5927 - RNA, 20 nt, synthetic construct
  source 1..20: mol_type = other RNA
gtaatacagtcccagtcgga

SEQ ID NO: 5928 - RNA, 20 nt, synthetic construct
  source 1..20: mol_type = other RNA
ctctctctcgccttccgact

SEQ ID NO: 5929 - RNA, 20 nt, synthetic construct
  source 1..20: mol_type = other RNA
gctctctctcgccttccgac

SEQ ID NO: 5930 - RNA, 20 nt, synthetic construct
  source 1..20: mol_type = other RNA
gaattgcagagaggggtaga

SEQ ID NO: 5931 - RNA, 20 nt, synthetic construct
  source 1..20: mol_type = other RNA
agaattgcagagaggggtag

SEQ ID NO: 5932 - RNA, 20 nt, synthetic construct
  source 1..20: mol_type = other RNA
ggcaggagaattgcagagag

SEQ ID NO: 5933 - RNA, 20 nt, synthetic construct
  source 1..20: mol_type = other RNA
tggcaggagaattgcagaga

SEQ ID NO: 5934 - RNA, 20 nt, synthetic construct
  source 1..20: mol_type = other RNA
gtggcaggagaattgcagag

SEQ ID NO: 5935 - RNA, 20 nt, synthetic construct
  source 1..20: mol_type = other RNA
aaggggcaaaactgggtggc

SEQ ID NO: 5936 - RNA, 20 nt, synthetic construct
  source 1..20: mol_type = other RNA
actcaaggggcaaaactggg

SEQ ID NO: 5937 - RNA, 20 nt, synthetic construct
  source 1..20: mol_type = other RNA
agaactcaaggggcaaaact

SEQ ID NO: 5938 - RNA, 20 nt, synthetic construct
  source 1..20: mol_type = other RNA
cagaactcaaggggcaaaac

SEQ ID NO: 5939 - RNA, 20 nt, synthetic construct
  source 1..20: mol_type = other RNA
cggttatggcagaactcaag

SEQ ID NO: 5940 - RNA, 20 nt, synthetic construct
  source 1..20: mol_type = other RNA
gcggttatggcagaactcaa

SEQ ID NO: 5941 - RNA, 20 nt, synthetic construct
  source 1..20: mol_type = other RNA
agttctgccataaccgcacc

SEQ ID NO: 5942 - RNA, 20 nt, synthetic construct
  source 1..20: mol_type = other RNA
ccataaccgcacctggagtg

SEQ ID NO: 5943 - RNA, 20 nt, synthetic construct
  source 1..20: mol_type = other RNA
cctcactccaggtgcggtta

SEQ ID NO: 5944 - RNA, 20 nt, synthetic construct
  source 1..20: mol_type = other RNA
ggagcgcctcactccaggtg

SEQ ID NO: 5945 - RNA, 20 nt, synthetic construct
  source 1..20: mol_type = other RNA
gacaaggagcgcctcactcc

SEQ ID NO: 5946 - RNA, 20 nt, synthetic construct
  source 1..20: mol_type = other RNA
agacgttgaggctagagaca

SEQ ID NO: 5947 - RNA, 20 nt, synthetic construct
  source 1..20: mol_type = other RNA
tgttgcaaaggaagacgttg

SEQ ID NO: 5948 - RNA, 20 nt, synthetic construct
  source 1..20: mol_type = other RNA
tcttcctttgcaacatgaga

SEQ ID NO: 5949 - RNA, 20 nt, synthetic construct
  source 1..20: mol_type = other RNA
cctttgcaacatgagaaggc

SEQ ID NO: 5950 - RNA, 20 nt, synthetic construct
  source 1..20: mol_type = other RNA
gcaacatgagaaggctggat

SEQ ID NO: 5951 - RNA, 20 nt, synthetic construct
  source 1..20: mol_type = other RNA
caacatgagaaggctggatt

SEQ ID NO: 5952 - RNA, 20 nt, synthetic construct
  source 1..20: mol_type = other RNA
tgacagttctgaaatgttag

SEQ ID NO: 5953 - RNA, 20 nt, synthetic construct
  source 1..20: mol_type = other RNA
cttcctgagcactgccagac

SEQ ID NO: 5954 - RNA, 20 nt, synthetic construct
  source 1..20: mol_type = other RNA
attcctgtctggcagtgctc

SEQ ID NO: 5955 - RNA, 20 nt, synthetic construct
  source 1..20: mol_type = other RNA
cactgccagacaggaatccc

SEQ ID NO: 5956 - RNA, 20 nt, synthetic construct
  source 1..20: mol_type = other RNA
atactccagggattcctgtc

SEQ ID NO: 5957 - RNA, 20 nt, synthetic construct
  source 1..20: mol_type = other RNA
gactctcttgacatactcca

SEQ ID NO: 5958 - RNA, 20 nt, synthetic construct
  source 1..20: mol_type = other RNA
tgactctcttgacatactcc

SEQ ID NO: 5959 - RNA, 20 nt, synthetic construct
  source 1..20: mol_type = other RNA
ataaaccttttcttgtttaa

SEQ ID NO: 5960 - RNA, 20 nt, synthetic construct
  source 1..20: mol_type = other RNA
accttttcttgtttaaaggt

SEQ ID NO: 5961 - RNA, 20 nt, synthetic construct
  source 1..20: mol_type = other RNA
tcctacctttaaacaagaaa

SEQ ID NO: 5962 - RNA, 20 nt, synthetic construct
  source 1..20: mol_type = other RNA
taaaggtaggacctccttct

SEQ ID NO: 5963 - RNA, 20 nt, synthetic construct
  source 1..20: mol_type = other RNA
atttgtttaagccaagaagg

SEQ ID NO: 5964 - RNA, 20 nt, synthetic construct
  source 1..20: mol_type = other RNA
cttggcttaaacaaatctca

SEQ ID NO: 5965 - RNA, 20 nt, synthetic construct
  source 1..20: mol_type = other RNA
gagatttgtttaagccaaga

SEQ ID NO: 5966 - RNA, 20 nt, synthetic construct
  source 1..20: mol_type = other RNA
ttaaacaaatctcaaggtgt

SEQ ID NO: 5967 - RNA, 20 nt, synthetic construct
  source 1..20: mol_type = other RNA
ggtgttggtctgcttcaaac

SEQ ID NO: 5968 - RNA, 20 nt, synthetic construct
  source 1..20: mol_type = other RNA
atctgtgaagtattagcaga

SEQ ID NO: 5969 - RNA, 20 nt, synthetic construct
  source 1..20: mol_type = other RNA
aagtattagcagacggcaag

SEQ ID NO: 5970 - RNA, 20 nt, synthetic construct
  source 1..20: mol_type = other RNA
acggcaagaggaatgtgttc

SEQ ID NO: 5971 - RNA, 20 nt, synthetic construct
  source 1..20: mol_type = other RNA
agaggaatgtgttcaggaag

SEQ ID NO: 5972 - RNA, 20 nt, synthetic construct
  source 1..20: mol_type = other RNA
aggaagaggacacttagctt

SEQ ID NO: 5973 - RNA, 20 nt, synthetic construct
  source 1..20: mol_type = other RNA
gaggacacttagcttaggtc

SEQ ID NO: 5974 - RNA, 20 nt, synthetic construct
  source 1..20: mol_type = other RNA
aggacacttagcttaggtct

SEQ ID NO: 5975 - RNA, 20 nt, synthetic construct
  source 1..20: mol_type = other RNA
ggacacttagcttaggtctg

SEQ ID NO: 5976 - RNA, 20 nt, synthetic construct
  source 1..20: mol_type = other RNA
gacacttagcttaggtctgg

SEQ ID NO: 5977 - RNA, 20 nt, synthetic construct
  source 1..20: mol_type = other RNA
gcttaggtctgggggaagca

SEQ ID NO: 5978 - RNA, 20 nt, synthetic construct
  source 1..20: mol_type = other RNA
cttaggtctgggggaagcat

SEQ ID NO: 5979 - RNA, 20 nt, synthetic construct
  source 1..20: mol_type = other RNA
ttaggtctgggggaagcatg

SEQ ID NO: 5980 - RNA, 20 nt, synthetic construct
  source 1..20: mol_type = other RNA
aagaagtcacaacacaactg

SEQ ID NO: 5981 - RNA, 20 nt, synthetic construct
  source 1..20: mol_type = other RNA
agaagtcacaacacaactgt

SEQ ID NO: 5982 - RNA, 20 nt, synthetic construct
  source 1..20: mol_type = other RNA
acaacacaactgtgggtgtc

SEQ ID NO: 5983 - RNA, 20 nt, synthetic construct
  source 1..20: mol_type = other RNA
gggtgtcaggctcttttctc

SEQ ID NO: 5984 - RNA, 20 nt, synthetic construct
  source 1..20: mol_type = other RNA
ggtgtcaggctcttttctct

SEQ ID NO: 5985 - RNA, 20 nt, synthetic construct
  source 1..20: mol_type = other RNA
gtgtcaggctcttttctctg

SEQ ID NO: 5986 - RNA, 20 nt, synthetic construct
  source 1..20: mol_type = other RNA
caccagagagtattcaagca

SEQ ID NO: 5987 - RNA, 20 nt, synthetic construct
  source 1..20: mol_type = other RNA
gagagtattcaagcatggat

SEQ ID NO: 5988 - RNA, 20 nt, synthetic construct
  source 1..20: mol_type = other RNA
atccatgcttgaatactctc

SEQ ID NO: 5989 - RNA, 20 nt, synthetic construct
  source 1..20: mol_type = other RNA
ggtagtccccatgcagccct

SEQ ID NO: 5990 - RNA, 20 nt, synthetic construct
  source 1..20: mol_type = other RNA
agtccccatgcagccctcgg

SEQ ID NO: 5991 - RNA, 20 nt, synthetic construct
  source 1..20: mol_type = other RNA
tttcctccgagggctgcatg

SEQ ID NO: 5992 - RNA, 20 nt, synthetic construct
  source 1..20: mol_type = other RNA
gtttcctccgagggctgcat

SEQ ID NO: 5993 - RNA, 20 nt, synthetic construct
  source 1..20: mol_type = other RNA
ggtttcctccgagggctgca

SEQ ID NO: 5994 - RNA, 20 nt, synthetic construct
  source 1..20: mol_type = other RNA
gcagcttcggtttcctccga

SEQ ID NO: 5995 - RNA, 20 nt, synthetic construct
  source 1..20: mol_type = other RNA
tgcagcttcggtttcctccg

SEQ ID NO: 5996 - RNA, 20 nt, synthetic construct
  source 1..20: mol_type = other RNA
agctgcaaatgcagcaatta

SEQ ID NO: 5997 - RNA, 20 nt, synthetic construct
  source 1..20: mol_type = other RNA
aattgctgcatttgcagctt

SEQ ID NO: 5998 - RNA, 20 nt, synthetic construct
  source 1..20: mol_type = other RNA
tatggcttacagcctgaaaa

SEQ ID NO: 5999 - RNA, 20 nt, synthetic construct
  source 1..20: mol_type = other RNA
tttggaatgtcaccattttc

SEQ ID NO: 6000 - RNA, 20 nt, synthetic construct
  source 1..20: mol_type = other RNA
attccaaaattgcatcttaa

SEQ ID NO: 6001 - RNA, 20 nt, synthetic construct
  source 1..20: mol_type = other RNA
ttccaaaattgcatcttaat

SEQ ID NO: 6002 - RNA, 20 nt, synthetic construct
  source 1..20: mol_type = other RNA
tacccattaagatgcaattt

SEQ ID NO: 6003 - RNA, 20 nt, synthetic construct
  source 1..20: mol_type = other RNA
catcttaatgggtaaaacat

SEQ ID NO: 6004 - RNA, 20 nt, synthetic construct
  source 1..20: mol_type = other RNA
cttaatgggtaaaacattgg

SEQ ID NO: 6005 - RNA, 20 nt, synthetic construct
  source 1..20: mol_type = other RNA
ggtaaaacattggtggagaa

SEQ ID NO: 6006 - RNA, 20 nt, synthetic construct
  source 1..20: mol_type = other RNA
gtaaaacattggtggagaaa

SEQ ID NO: 6007 - RNA, 20 nt, synthetic construct
  source 1..20: mol_type = other RNA
ggcagcagaagatccccaca

SEQ ID NO: 6008 - RNA, 20 nt, synthetic construct
  source 1..20: mol_type = other RNA
agatccccacaaggtccttc

SEQ ID NO: 6009 - RNA, 20 nt, synthetic construct
  source 1..20: mol_type = other RNA
ccacaaggtccttcaggtac

SEQ ID NO: 6010 - RNA, 20 nt, synthetic construct
  source 1..20: mol_type = other RNA
tgtacctgaaggaccttgtg

SEQ ID NO: 6011 - RNA, 20 nt, synthetic construct
  source 1..20: mol_type = other RNA
ctgtacctgaaggaccttgt

SEQ ID NO: 6012 - RNA, 20 nt, synthetic construct
  source 1..20: mol_type = other RNA
cctgtacctgaaggaccttg

SEQ ID NO: 6013 - RNA, 20 nt, synthetic construct
  source 1..20: mol_type = other RNA
tgggagatgcctgtacctga

SEQ ID NO: 6014 - RNA, 20 nt, synthetic construct
  source 1..20: mol_type = other RNA
cccactgctcagagtcctgc

SEQ ID NO: 6015 - RNA, 20 nt, synthetic construct
  source 1..20: mol_type = other RNA
ccactgctcagagtcctgct

SEQ ID NO: 6016 - RNA, 20 nt, synthetic construct
  source 1..20: mol_type = other RNA
cactgctcagagtcctgctg

SEQ ID NO: 6017 - RNA, 20 nt, synthetic construct
  source 1..20: mol_type = other RNA
actgctcagagtcctgctgg

SEQ ID NO: 6018 - RNA, 20 nt, synthetic construct
  source 1..20: mol_type = other RNA
ccagcaggactctgagcagt

SEQ ID NO: 6019 - RNA, 20 nt, synthetic construct
  source 1..20: mol_type = other RNA
cccagcaggactctgagcag

SEQ ID NO: 6020 - RNA, 20 nt, synthetic construct
  source 1..20: mol_type = other RNA
gggacttggggacccccagc

SEQ ID NO: 6021 - RNA, 20 nt, synthetic construct
  source 1..20: mol_type = other RNA
ttcttcttgtttgggacttg

SEQ ID NO: 6022 - RNA, 20 nt, synthetic construct
  source 1..20: mol_type = other RNA
cttcttcttgtttgggactt

SEQ ID NO: 6023 - RNA, 20 nt, synthetic construct
  source 1..20: mol_type = other RNA
gcttcttcttgtttgggact

SEQ ID NO: 6024 - RNA, 20 nt, synthetic construct
  source 1..20: mol_type = other RNA
ctctctgcttcttcttgttt

SEQ ID NO: 6025 - RNA, 20 nt, synthetic construct
  source 1..20: mol_type = other RNA
gctctctgcttcttcttgtt

SEQ ID NO: 6026 - RNA, 20 nt, synthetic construct
  source 1..20: mol_type = other RNA
agagcagagttcacctcttc

SEQ ID NO: 6027 - RNA, 20 nt, synthetic construct
  source 1..20: mol_type = other RNA
tttatcttaagctcctgaag

SEQ ID NO: 6028 - RNA, 20 nt, synthetic construct
  source 1..20: mol_type = other RNA
acaagttcatgcagcagaca

SEQ ID NO: 6029 - RNA, 20 nt, synthetic construct
  source 1..20: mol_type = other RNA
gttcatgcagcagacacggc

SEQ ID NO: 6030 - RNA, 20 nt, synthetic construct
  source 1..20: mol_type = other RNA
agtgcagatggatgttgggt

SEQ ID NO: 6031 - RNA, 20 nt, synthetic construct
  source 1..20: mol_type = other RNA
aagtgcagatggatgttggg

SEQ ID NO: 6032 - RNA, 20 nt, synthetic construct
  source 1..20: mol_type = other RNA
gacaagtgcagatggatgtt

SEQ ID NO: 6033 - RNA, 20 nt, synthetic construct
  source 1..20: mol_type = other RNA
ggacaagtgcagatggatgt

SEQ ID NO: 6034 - RNA, 20 nt, synthetic construct
  source 1..20: mol_type = other RNA
ctatcaaggacaagtgcaga

SEQ ID NO: 6035 - RNA, 20 nt, synthetic construct
  source 1..20: mol_type = other RNA
ttgatagcaaaacctgagtc

SEQ ID NO: 6036 - RNA, 20 nt, synthetic construct
  source 1..20: mol_type = other RNA
agactcaggttttgctatca

SEQ ID NO: 6037 - RNA, 20 nt, synthetic construct
  source 1..20: mol_type = other RNA
agcaaaacctgagtctggtt

SEQ ID NO: 6038 - RNA, 20 nt, synthetic construct
  source 1..20: mol_type = other RNA
gcaaaacctgagtctggttt

SEQ ID NO: 6039 - RNA, 20 nt, synthetic construct
  source 1..20: mol_type = other RNA
caaaacctgagtctggtttg

SEQ ID NO: 6040 - RNA, 20 nt, synthetic construct
  source 1..20: mol_type = other RNA
gacttccccaaaccagactc

SEQ ID NO: 6041 - RNA, 20 nt, synthetic construct
  source 1..20: mol_type = other RNA
aaaatacagttatgtcagct

SEQ ID NO: 6042 - RNA, 20 nt, synthetic construct
  source 1..20: mol_type = other RNA
gaaaatacagttatgtcagc

SEQ ID NO: 6043 - RNA, 20 nt, synthetic construct
  source 1..20: mol_type = other RNA
gtctctcttattgcaagaac

SEQ ID NO: 6044 - RNA, 20 nt, synthetic construct
  source 1..20: mol_type = other RNA
tctctcttattgcaagaact

SEQ ID NO: 6045 - RNA, 20 nt, synthetic construct
  source 1..20: mol_type = other RNA
ctgggcatatgacttagttc

SEQ ID NO: 6046 - RNA, 20 nt, synthetic construct
  source 1..20: mol_type = other RNA
gacataaacgggtgtcttat

SEQ ID NO: 6047 - RNA, 20 nt, synthetic construct
  source 1..20: mol_type = other RNA
gacacccgtttatgtcagtc

SEQ ID NO: 6048 - RNA, 20 nt, synthetic construct
  source 1..20: mol_type = other RNA
aaatcctgactgacataaac

SEQ ID NO: 6049 - RNA, 20 nt, synthetic construct
  source 1..20: mol_type = other RNA
gaaatcctgactgacataaa

SEQ ID NO: 6050 - RNA, 20 nt, synthetic construct
  source 1..20: mol_type = other RNA
aaggggtggtgtctactgca

SEQ ID NO: 6051 - RNA, 20 nt, synthetic construct
  source 1..20: mol_type = other RNA
gaaggggtggtgtctactgc

SEQ ID NO: 6052 - RNA, 20 nt, synthetic construct
  source 1..20: mol_type = other RNA
tagacaccaccccttcctct

SEQ ID NO: 6053 - RNA, 20 nt, synthetic construct
  source 1..20: mol_type = other RNA
aagtgacctagaggaagggg

SEQ ID NO: 6054 - RNA, 20 nt, synthetic construct
  source 1..20: mol_type = other RNA
agaaagtgacctagaggaag

SEQ ID NO: 6055 - RNA, 20 nt, synthetic construct
  source 1..20: mol_type = other RNA
aagaaagtgacctagaggaa

SEQ ID NO: 6056 - RNA, 20 nt, synthetic construct
  source 1..20: mol_type = other RNA
gaagaaagtgacctagagga

SEQ ID NO: 6057 - RNA, 20 nt, synthetic construct
  source 1..20: mol_type = other RNA
ggaagaagaaagtgacctag

SEQ ID NO: 6058 - RNA, 20 nt, synthetic construct
  source 1..20: mol_type = other RNA
tttcttcttcctgtccagaa

SEQ ID NO: 6059 - RNA, 20 nt, synthetic construct
  source 1..20: mol_type = other RNA
cttcttcctgtccagaaagg

SEQ ID NO: 6060 - RNA, 20 nt, synthetic construct
  source 1..20: mol_type = other RNA
gcttctccacctttctggac

SEQ ID NO: 6061 - RNA, 20 nt, synthetic construct
  source 1..20: mol_type = other RNA
tgatggcttctccacctttc

SEQ ID NO: 6062 - RNA, 20 nt, synthetic construct
  source 1..20: mol_type = other RNA
gagaagccatcatcaatttt

SEQ ID NO: 6063 - RNA, 20 nt, synthetic construct
  source 1..20: mol_type = other RNA
tttgctcctaaaattgatga

SEQ ID NO: 6064 - RNA, 20 nt, synthetic construct
  source 1..20: mol_type = other RNA
caaaagccacagactaaagt

SEQ ID NO: 6065 - RNA, 20 nt, synthetic construct
  source 1..20: mol_type = other RNA
gacttgccaactttagtctg

SEQ ID NO: 6066 - RNA, 20 nt, synthetic construct
  source 1..20: mol_type = other RNA
ttggcaagtctgaagttaaa

SEQ ID NO: 6067 - RNA, 20 nt, synthetic construct
  source 1..20: mol_type = other RNA
gcaagtctgaagttaaaagg

SEQ ID NO: 6068 - RNA, 20 nt, synthetic construct
  source 1..20: mol_type = other RNA
tctgaagttaaaaggaggct

SEQ ID NO: 6069 - RNA, 20 nt, synthetic construct
  source 1..20: mol_type = other RNA
gttatatgaagcagtcatca

SEQ ID NO: 6070 - RNA, 20 nt, synthetic construct
  source 1..20: mol_type = other RNA
tcatataaccctaccatctt

SEQ ID NO: 6071 - RNA, 20 nt, synthetic construct
  source 1..20: mol_type = other RNA
aggatggtccaaagatggta

SEQ ID NO: 6072 - RNA, 20 nt, synthetic construct
  source 1..20: mol_type = other RNA
taggatggtccaaagatggt

SEQ ID NO: 6073 - RNA, 20 nt, synthetic construct
  source 1..20: mol_type = other RNA
tgggtaggatggtccaaaga

SEQ ID NO: 6074 - RNA, 20 nt, synthetic construct
  source 1..20: mol_type = other RNA
tggaccatcctacccagatc

SEQ ID NO: 6075 - RNA, 20 nt, synthetic construct
  source 1..20: mol_type = other RNA
aagtccagatctgggtagga

SEQ ID NO: 6076 - RNA, 20 nt, synthetic construct
  source 1..20: mol_type = other RNA
ctaaaagtccagatctgggt

SEQ ID NO: 6077 - RNA, 20 nt, synthetic construct
  source 1..20: mol_type = other RNA
gttcctaaaagtccagatct

SEQ ID NO: 6078 - RNA, 20 nt, synthetic construct
  source 1..20: mol_type = other RNA
tgttcctaaaagtccagatc

SEQ ID NO: 6079 - RNA, 20 nt, synthetic construct
  source 1..20: mol_type = other RNA
gaacaaaataagaccctatg

SEQ ID NO: 6080 - RNA, 20 nt, synthetic construct
  source 1..20: mol_type = other RNA
atgtggctaagccactctag

SEQ ID NO: 6081 - RNA, 20 nt, synthetic construct
  source 1..20: mol_type = other RNA
tagagtggcttagccacata

SEQ ID NO: 6082 - RNA, 20 nt, synthetic construct
  source 1..20: mol_type = other RNA
ctagagtggcttagccacat

SEQ ID NO: 6083 - RNA, 20 nt, synthetic construct
  source 1..20: mol_type = other RNA
tattcaaaacaccgctagag

SEQ ID NO: 6084 - RNA, 20 nt, synthetic construct
  source 1..20: mol_type = other RNA
gggactgtgacttctctaat

SEQ ID NO: 6085 - RNA, 20 nt, synthetic construct
  source 1..20: mol_type = other RNA
agggactgtgacttctctaa

SEQ ID NO: 6086 - RNA, 20 nt, synthetic construct
  source 1..20: mol_type = other RNA
aatgtgcggggcacatttaa

SEQ ID NO: 6087 - RNA, 20 nt, synthetic construct
  source 1..20: mol_type = other RNA
caatgtgcggggcacattta

SEQ ID NO: 6088 - RNA, 20 nt, synthetic construct
  source 1..20: mol_type = other RNA
gcacattgccgtgtatagtc

SEQ ID NO: 6089 - RNA, 20 nt, synthetic construct
  source 1..20: mol_type = other RNA
actatacacggcaatgtgcg

SEQ ID NO: 6090 - RNA, 20 nt, synthetic construct
  source 1..20: mol_type = other RNA
gactatacacggcaatgtgc

SEQ ID NO: 6091 - RNA, 20 nt, synthetic construct
  source 1..20: mol_type = other RNA
tgactatacacggcaatgtg

SEQ ID NO: 6092 - RNA, 20 nt, synthetic construct
  source 1..20: mol_type = other RNA
ctggtagtcctgactataca

SEQ ID NO: 6093 - RNA, 20 nt, synthetic construct
  source 1..20: mol_type = other RNA
ggcatataggctgggatatc

SEQ ID NO: 6094 - RNA, 20 nt, synthetic construct
  source 1..20: mol_type = other RNA
tcccagcctatatgccccaa

SEQ ID NO: 6095 - RNA, 20 nt, synthetic construct
  source 1..20: mol_type = other RNA
cccagcctatatgccccaat

SEQ ID NO: 6096 - RNA, 20 nt, synthetic construct
  source 1..20: mol_type = other RNA
ccagcctatatgccccaatg

SEQ ID NO: 6097 - RNA, 20 nt, synthetic construct
  source 1..20: mol_type = other RNA
cagcctatatgccccaatgg

SEQ ID NO: 6098 - RNA, 20 nt, synthetic construct
  source 1..20: mol_type = other RNA
cccattggggcatataggct

SEQ ID NO: 6099 - RNA, 20 nt, synthetic construct
  source 1..20: mol_type = other RNA
ccccattggggcatataggc

SEQ ID NO: 6100 - RNA, 20 nt, synthetic construct
  source 1..20: mol_type = other RNA
ctgcccccattggggcatat

SEQ ID NO: 6101 - RNA, 20 nt, synthetic construct
  source 1..20: mol_type = other RNA
tggcagtgctgcccccattg

SEQ ID NO: 6102 - RNA, 20 nt, synthetic construct
  source 1..20: mol_type = other RNA
ttggcagtgctgcccccatt

SEQ ID NO: 6103 - RNA, 20 nt, synthetic construct
  source 1..20: mol_type = other RNA
tttggcagtgctgcccccat

SEQ ID NO: 6104 - RNA, 20 nt, synthetic construct
  source 1..20: mol_type = other RNA
gtaaatcacacttaattctt

SEQ ID NO: 6105 - RNA, 20 nt, synthetic construct
  source 1..20: mol_type = other RNA
acatgtaaggaagtaatcac

SEQ ID NO: 6106 - RNA, 20 nt, synthetic construct
  source 1..20: mol_type = other RNA
agtagtcaagattacatgta

SEQ ID NO: 6107 - RNA, 20 nt, synthetic construct
  source 1..20: mol_type = other RNA
ttaattaacttgcttacaat

SEQ ID NO: 6108 - RNA, 20 nt, synthetic construct
  source 1..20: mol_type = other RNA
tgtctgaagactgattaatc

SEQ ID NO: 6109 - RNA, 20 nt, synthetic construct
  source 1..20: mol_type = other RNA
atggaatattcaaaaaatgc

SEQ ID NO: 6110 - RNA, 20 nt, synthetic construct
  source 1..20: mol_type = other RNA
aaataaagaaacaaataata

SEQ ID NO: 6111 - RNA, 20 nt, synthetic construct
  source 1..20: mol_type = other RNA
tttcatgttatttgttaacc

SEQ ID NO: 6112 - RNA, 20 nt, synthetic construct
  source 1..20: mol_type = other RNA
gtagttggtttcttggaaga

SEQ ID NO: 6113 - RNA, 20 nt, synthetic construct
  source 1..20: mol_type = other RNA
tagttggtttcttggaagaa

SEQ ID NO: 6114 - RNA, 20 nt, synthetic construct
  source 1..20: mol_type = other RNA
cttcataaagaagctagagc

SEQ ID NO: 6115 - RNA, 20 nt, synthetic construct
  source 1..20: mol_type = other RNA
agctagagctggccacaaga

SEQ ID NO: 6116 - RNA, 20 nt, synthetic construct
  source 1..20: mol_type = other RNA
tgtgggcattttccttcttg

SEQ ID NO: 6117 - RNA, 20 nt, synthetic construct
  source 1..20: mol_type = other RNA
gaaaatgcccacaacaagat

SEQ ID NO: 6118 - RNA, 20 nt, synthetic construct
  source 1..20: mol_type = other RNA
aatgcccacaacaagatagg

SEQ ID NO: 6119 - RNA, 20 nt, synthetic construct
  source 1..20: mol_type = other RNA
cccacaacaagataggaggc

SEQ ID NO: 6120 - RNA, 20 nt, synthetic construct
  source 1..20: mol_type = other RNA
cctgcctcctatcttgttgt

SEQ ID NO: 6121 - RNA, 20 nt, synthetic construct
  source 1..20: mol_type = other RNA
tcctgcctcctatcttgttg

SEQ ID NO: 6122 - RNA, 20 nt, synthetic construct
  source 1..20: mol_type = other RNA
gataggaggcaggaaacccc

SEQ ID NO: 6123 - RNA, 20 nt, synthetic construct
  source 1..20: mol_type = other RNA
taggtatctttcttttccag

SEQ ID NO: 6124 - RNA, 20 nt, synthetic construct
  source 1..20: mol_type = other RNA
gtaggtatctttcttttcca

SEQ ID NO: 6125 - RNA, 20 nt, synthetic construct
  source 1..20: mol_type = other RNA
ggtaggtatctttcttttcc

SEQ ID NO: 6126 - RNA, 20 nt, synthetic construct
  source 1..20: mol_type = other RNA
atacctacctgctagttctc

SEQ ID NO: 6127 - RNA, 20 nt, synthetic construct
  source 1..20: mol_type = other RNA
tacctacctgctagttctca

SEQ ID NO: 6128 - RNA, 20 nt, synthetic construct
  source 1..20: mol_type = other RNA
cctgctagttctcagggaag

SEQ ID NO: 6129 - RNA, 20 nt, synthetic construct
  source 1..20: mol_type = other RNA
ttccctgagaactagcaggt

SEQ ID NO: 6130 - RNA, 20 nt, synthetic construct
  source 1..20: mol_type = other RNA
ctagttctcagggaagaggc

SEQ ID NO: 6131 - RNA, 20 nt, synthetic construct
  source 1..20: mol_type = other RNA
cctcttccctgagaactagc

SEQ ID NO: 6132 - RNA, 20 nt, synthetic construct
  source 1..20: mol_type = other RNA
ctcagggaagaggctgggcc

SEQ ID NO: 6133 - RNA, 20 nt, synthetic construct
  source 1..20: mol_type = other RNA
ggaagaggctgggccaggca

SEQ ID NO: 6134 - RNA, 20 nt, synthetic construct
  source 1..20: mol_type = other RNA
agaggctgggccaggcatgg

SEQ ID NO: 6135 - RNA, 20 nt, synthetic construct
  source 1..20: mol_type = other RNA
caggcatgagccaccatgcc

SEQ ID NO: 6136 - RNA, 20 nt, synthetic construct
  source 1..20: mol_type = other RNA
tgtaatcccagtactttgag

SEQ ID NO: 6137 - RNA, 20 nt, synthetic construct
  source 1..20: mol_type = other RNA
tctcaaagtactgggattac

SEQ ID NO: 6138 - RNA, 20 nt, synthetic construct
  source 1..20: mol_type = other RNA
cccagtactttgagaggctg

SEQ ID NO: 6139 - RNA, 20 nt, synthetic construct
  source 1..20: mol_type = other RNA
gtactttgagaggctgaggc

SEQ ID NO: 6140 - RNA, 20 nt, synthetic construct
  source 1..20: mol_type = other RNA
cctcagcctctcaaagtact

SEQ ID NO: 6141 - RNA, 20 nt, synthetic construct
  source 1..20: mol_type = other RNA
gcctcagcctctcaaagtac

SEQ ID NO: 6142 - RNA, 20 nt, synthetic construct
  source 1..20: mol_type = other RNA
ctttgagaggctgaggctgg

SEQ ID NO: 6143 - RNA, 20 nt, synthetic construct
  source 1..20: mol_type = other RNA
gctggaggatcacttaagcc

SEQ ID NO: 6144 - RNA, 20 nt, synthetic construct
  source 1..20: mol_type = other RNA
ccaggagttcaagacaagcc

SEQ ID NO: 6145 - RNA, 20 nt, synthetic construct
  source 1..20: mol_type = other RNA
caggagttcaagacaagcct

SEQ ID NO: 6146 - RNA, 20 nt, synthetic construct
  source 1..20: mol_type = other RNA
ccaggcttgtcttgaactcc

SEQ ID NO: 6147 - RNA, 20 nt, synthetic construct
  source 1..20: mol_type = other RNA
caagacaagcctgggcgaca

SEQ ID NO: 6148 - RNA, 20 nt, synthetic construct
  source 1..20: mol_type = other RNA
agggtctcaccatgtcgccc

SEQ ID NO: 6149 - RNA, 20 nt, synthetic construct
  source 1..20: mol_type = other RNA
ttttattttttgtagggaca

SEQ ID NO: 6150 - RNA, 20 nt, synthetic construct
  source 1..20: mol_type = other RNA
tttttattttttgtagggac

SEQ ID NO: 6151 - RNA, 20 nt, synthetic construct
  source 1..20: mol_type = other RNA
acaaaaaataaaaaattagc

SEQ ID NO: 6152 - RNA, 20 nt, synthetic construct
  source 1..20: mol_type = other RNA
ctaattttttattttttgta

SEQ ID NO: 6153 - RNA, 20 nt, synthetic construct
  source 1..20: mol_type = other RNA
gctaattttttattttttgt

SEQ ID NO: 6154 - RNA, 20 nt, synthetic construct
  source 1..20: mol_type = other RNA
aataaaaaattagctggcca

SEQ ID NO: 6155 - RNA, 20 nt, synthetic construct
  source 1..20: mol_type = other RNA
aaaaaattagctggccatgg

SEQ ID NO: 6156 - RNA, 20 nt, synthetic construct
  source 1..20: mol_type = other RNA
actacaagtgtgtgccacca

SEQ ID NO: 6157 - RNA, 20 nt, synthetic construct
  source 1..20: mol_type = other RNA
tgtagtcccagctactcaag

SEQ ID NO: 6158 - RNA, 20 nt, synthetic construct
  source 1..20: mol_type = other RNA
cccagctactcaagaggctg

SEQ ID NO: 6159 - RNA, 20 nt, synthetic construct
  source 1..20: mol_type = other RNA
agctactcaagaggctgagg

SEQ ID NO: 6160 - RNA, 20 nt, synthetic construct
  source 1..20: mol_type = other RNA
gctactcaagaggctgaggt

SEQ ID NO: 6161 - RNA, 20 nt, synthetic construct
  source 1..20: mol_type = other RNA
cctcagcctcttgagtagct

SEQ ID NO: 6162 - RNA, 20 nt, synthetic construct
  source 1..20: mol_type = other RNA
acctcagcctcttgagtagc

SEQ ID NO: 6163 - RNA, 20 nt, synthetic construct
  source 1..20: mol_type = other RNA
actcaagaggctgaggtggg

SEQ ID NO: 6164 - RNA, 20 nt, synthetic construct
  source 1..20: mol_type = other RNA
tcacttgagctccaaagtca

SEQ ID NO: 6165 - RNA, 20 nt, synthetic construct
  source 1..20: mol_type = other RNA
gctcactgcagccttgactt

SEQ ID NO: 6166 - RNA, 20 nt, synthetic construct
  source 1..20: mol_type = other RNA
gatattttagttacgttaag

SEQ ID NO: 6167 - RNA, 20 nt, synthetic construct
  source 1..20: mol_type = other RNA
tatctattctgatgagattc

SEQ ID NO: 6168 - RNA, 20 nt, synthetic construct
  source 1..20: mol_type = other RNA
ttcgaggggaaaagtcattt

SEQ ID NO: 6169 - RNA, 20 nt, synthetic construct
  source 1..20: mol_type = other RNA
attcgaggggaaaagtcatt

SEQ ID NO: 6170 - RNA, 20 nt, synthetic construct
  source 1..20: mol_type = other RNA
gacttttcccctcgaatcat

SEQ ID NO: 6171 - RNA, 20 nt, synthetic construct
  source 1..20: mol_type = other RNA
gcagtttcctatgattcgag

SEQ ID NO: 6172 - RNA, 20 nt, synthetic construct
  source 1..20: mol_type = other RNA
tgcagtttcctatgattcga

SEQ ID NO: 6173 - RNA, 20 nt, synthetic construct
  source 1..20: mol_type = other RNA
ctgcagtttcctatgattcg

SEQ ID NO: 6174 - RNA, 20 nt, synthetic construct
  source 1..20: mol_type = other RNA
tacctgcttgccagttactc

SEQ ID NO: 6175 - RNA, 20 nt, synthetic construct
  source 1..20: mol_type = other RNA
atccggagtaactggcaagc

SEQ ID NO: 6176 - RNA, 20 nt, synthetic construct
  source 1..20: mol_type = other RNA
aagcatcaatccggagtaac

SEQ ID NO: 6177 - RNA, 20 nt, synthetic construct
  source 1..20: mol_type = other RNA
tacatcgggaagcatcaatc

SEQ ID NO: 6178 - RNA, 20 nt, synthetic construct
  source 1..20: mol_type = other RNA
atgcttcccgatgtaaacaa

SEQ ID NO: 6179 - RNA, 20 nt, synthetic construct
  source 1..20: mol_type = other RNA
gatcagccattgtttacatc

SEQ ID NO: 6180 - RNA, 20 nt, synthetic construct
  source 1..20: mol_type = other RNA
cgatcagccattgtttacat

SEQ ID NO: 6181 - RNA, 20 nt, synthetic construct
  source 1..20: mol_type = other RNA
ttctgcaaaacaaaagcgat

SEQ ID NO: 6182 - RNA, 20 nt, synthetic construct
  source 1..20: mol_type = other RNA
tctgcaaaacaaaagcgatt

SEQ ID NO: 6183 - RNA, 20 nt, synthetic construct
  source 1..20: mol_type = other RNA
acaaaagcgattgggtattt

SEQ ID NO: 6184 - RNA, 20 nt, synthetic construct
  source 1..20: mol_type = other RNA
catcagtttagtagtttccc

SEQ ID NO: 6185 - RNA, 20 nt, synthetic construct
  source 1..20: mol_type = other RNA
gagttataggacatttgcca

SEQ ID NO: 6186 - RNA, 20 nt, synthetic construct
  source 1..20: mol_type = other RNA
agagttataggacatttgcc

SEQ ID NO: 6187 - RNA, 20 nt, synthetic construct
  source 1..20: mol_type = other RNA
acacacacacacagagttat

SEQ ID NO: 6188 - RNA, 20 nt, synthetic construct
  source 1..20: mol_type = other RNA
tgcccatgctccgctggtca

SEQ ID NO: 6189 - RNA, 20 nt, synthetic construct
  source 1..20: mol_type = other RNA
gtgcccatgctccgctggtc

SEQ ID NO: 6190 - RNA, 20 nt, synthetic construct
  source 1..20: mol_type = other RNA
tagctgtgcccatgctccgc

SEQ ID NO: 6191 - RNA, 20 nt, synthetic construct
  source 1..20: mol_type = other RNA
tacttagagcgccacccttc

SEQ ID NO: 6192 - RNA, 20 nt, synthetic construct
  source 1..20: mol_type = other RNA
cacccttcaggacacaaagt

SEQ ID NO: 6193 - RNA, 20 nt, synthetic construct
  source 1..20: mol_type = other RNA
acccttcaggacacaaagtc

SEQ ID NO: 6194 - RNA, 20 nt, synthetic construct
  source 1..20: mol_type = other RNA
cccttcaggacacaaagtcg

SEQ ID NO: 6195 - RNA, 20 nt, synthetic construct
  source 1..20: mol_type = other RNA
cgactttgtgtcctgaaggg

SEQ ID NO: 6196 - RNA, 20 nt, synthetic construct
  source 1..20: mol_type = other RNA
ccccgactttgtgtcctgaa

SEQ ID NO: 6197 - RNA, 20 nt, synthetic construct
  source 1..20: mol_type = other RNA
gccccgactttgtgtcctga

SEQ ID NO: 6198 - RNA, 20 nt, synthetic construct
  source 1..20: mol_type = other RNA
gtcggggctacctctcttcc

SEQ ID NO: 6199 - RNA, 20 nt, synthetic construct
  source 1..20: mol_type = other RNA
ggctacctctcttccaggca

SEQ ID NO: 6200 - RNA, 20 nt, synthetic construct
  source 1..20: mol_type = other RNA
ggatgccttgcctggaagag

SEQ ID NO: 6201 - RNA, 20 nt, synthetic construct
  source 1..20: mol_type = other RNA
ttccaggcaaggcatcctag

SEQ ID NO: 6202 - RNA, 20 nt, synthetic construct
  source 1..20: mol_type = other RNA
tccaggcaaggcatcctaga

SEQ ID NO: 6203 - RNA, 20 nt, synthetic construct
  source 1..20: mol_type = other RNA
gccctctaggatgccttgcc

SEQ ID NO: 6204 - RNA, 20 nt, synthetic construct
  source 1..20: mol_type = other RNA
ggagggtgtgcgggccctct

SEQ ID NO: 6205 - RNA, 20 nt, synthetic construct
  source 1..20: mol_type = other RNA
gatcaaactggagggtgtgc

SEQ ID NO: 6206 - RNA, 20 nt, synthetic construct
  source 1..20: mol_type = other RNA
agatcaaactggagggtgtg

SEQ ID NO: 6207 - RNA, 20 nt, synthetic construct
  source 1..20: mol_type = other RNA
agaggtaagatcaaactgga

SEQ ID NO: 6208 - RNA, 20 nt, synthetic construct
  source 1..20: mol_type = other RNA
gagaggtaagatcaaactgg

SEQ ID NO: 6209 - RNA, 20 nt, synthetic construct
  source 1..20: mol_type = other RNA
gctgagaggtaagatcaaac

SEQ ID NO: 6210 - RNA, 20 nt, synthetic construct
  source 1..20: mol_type = other RNA
gaaaaggaacgggagctgag

SEQ ID NO: 6211 - RNA, 20 nt, synthetic construct
  source 1..20: mol_type = other RNA
gggagagaaagaaaaggaac

SEQ ID NO: 6212 - RNA, 20 nt, synthetic construct
  source 1..20: mol_type = other RNA
ggggagagaaagaaaaggaa

SEQ ID NO: 6213 - RNA, 20 nt, synthetic construct
  source 1..20: mol_type = other RNA
ttactggggagagaaagaaa

SEQ ID NO: 6214 - RNA, 20 nt, synthetic construct
  source 1..20: mol_type = other RNA
agacgttcaacgacttactg

SEQ ID NO: 6215 - RNA, 20 nt, synthetic construct
  source 1..20: mol_type = other RNA
aagacgttcaacgacttact

SEQ ID NO: 6216 - RNA, 20 nt, synthetic construct
  source 1..20: mol_type = other RNA
aaagacgttcaacgacttac

SEQ ID NO: 6217 - RNA, 20 nt, synthetic construct
  source 1..20: mol_type = other RNA
cgttgaacgtctttcttctg

SEQ ID NO: 6218 - RNA, 20 nt, synthetic construct
  source 1..20: mol_type = other RNA
ctttcttctgaggctgagcg

SEQ ID NO: 6219 - RNA, 20 nt, synthetic construct
  source 1..20: mol_type = other RNA
gcgtggagctctcttctcgc

SEQ ID NO: 6220 - RNA, 20 nt, synthetic construct
  source 1..20: mol_type = other RNA
tcgctggcgagctttctgaa

SEQ ID NO: 6221 - RNA, 20 nt, synthetic construct
  source 1..20: mol_type = other RNA
atggcactttctgtacaaac

SEQ ID NO: 6222 - RNA, 20 nt, synthetic construct
  source 1..20: mol_type = other RNA
acaaacaggaagagcatgtg

SEQ ID NO: 6223 - RNA, 20 nt, synthetic construct
  source 1..20: mol_type = other RNA
tggtcacaacccaagtgtgc

SEQ ID NO: 6224 - RNA, 20 nt, synthetic construct
  source 1..20: mol_type = other RNA
aagtgtgcaggtgttgatag

SEQ ID NO: 6225 - RNA, 20 nt, synthetic construct
  source 1..20: mol_type = other RNA
ctatcaacacctgcacactt

SEQ ID NO: 6226 - RNA, 20 nt, synthetic construct
  source 1..20: mol_type = other RNA
tctatcaacacctgcacact

SEQ ID NO: 6227 - RNA, 20 nt, synthetic construct
  source 1..20: mol_type = other RNA
tgatagaggatgtgaaagtg

SEQ ID NO: 6228 - RNA, 20 nt, synthetic construct
  source 1..20: mol_type = other RNA
tagaggatgtgaaagtgtgg

SEQ ID NO: 6229 - RNA, 20 nt, synthetic construct
  source 1..20: mol_type = other RNA
gactaaaccagatacccaac

SEQ ID NO: 6230 - RNA, 20 nt, synthetic construct
  source 1..20: mol_type = other RNA
gagttggccggttgggtatc

SEQ ID NO: 6231 - RNA, 20 nt, synthetic construct
  source 1..20: mol_type = other RNA
aaccggccaactctcacttg

SEQ ID NO: 6232 - RNA, 20 nt, synthetic construct
  source 1..20: mol_type = other RNA
caagtgagagttggccggtt

SEQ ID NO: 6233 - RNA, 20 nt, synthetic construct
  source 1..20: mol_type = other RNA
acaagtgagagttggccggt

SEQ ID NO: 6234 - RNA, 20 nt, synthetic construct
  source 1..20: mol_type = other RNA
ggccaactctcacttgtggc

SEQ ID NO: 6235 - RNA, 20 nt, synthetic construct
  source 1..20: mol_type = other RNA
gccaactctcacttgtggca

SEQ ID NO: 6236 - RNA, 20 nt, synthetic construct
  source 1..20: mol_type = other RNA
tgccacaagtgagagttggc

SEQ ID NO: 6237 - RNA, 20 nt, synthetic construct
  source 1..20: mol_type = other RNA
ctctcacttgtggcagggcc

SEQ ID NO: 6238 - RNA, 20 nt, synthetic construct
  source 1..20: mol_type = other RNA
gccctgccacaagtgagagt

SEQ ID NO: 6239 - RNA, 20 nt, synthetic construct
  source 1..20: mol_type = other RNA
gcagggcctggtctaccaga

SEQ ID NO: 6240 - RNA, 20 nt, synthetic construct
  source 1..20: mol_type = other RNA
ggcctggtctaccagaaggc

SEQ ID NO: 6241 - RNA, 20 nt, synthetic construct
  source 1..20: mol_type = other RNA
tctaccagaaggctggaagc

SEQ ID NO: 6242 - RNA, 20 nt, synthetic construct
  source 1..20: mol_type = other RNA
gaaggctggaagcaggaacc

SEQ ID NO: 6243 - RNA, 20 nt, synthetic construct
  source 1..20: mol_type = other RNA
ggttcctgcttccagccttc

SEQ ID NO: 6244 - RNA, 20 nt, synthetic construct
  source 1..20: mol_type = other RNA
caggaacctggactctactc

SEQ ID NO: 6245 - RNA, 20 nt, synthetic construct
  source 1..20: mol_type = other RNA
aggaacctggactctactct

SEQ ID NO: 6246 - RNA, 20 nt, synthetic construct
  source 1..20: mol_type = other RNA
ggaacctggactctactctg

SEQ ID NO: 6247 - RNA, 20 nt, synthetic construct
  source 1..20: mol_type = other RNA
gtctccccagagtagagtcc

SEQ ID NO: 6248 - RNA, 20 nt, synthetic construct
  source 1..20: mol_type = other RNA
agaccaactgacaaaagcag

SEQ ID NO: 6249 - RNA, 20 nt, synthetic construct
  source 1..20: mol_type = other RNA
caactgacaaaagcagagga

SEQ ID NO: 6250 - RNA, 20 nt, synthetic construct
  source 1..20: mol_type = other RNA
ctgacaaaagcagaggatgg

SEQ ID NO: 6251 - RNA, 20 nt, synthetic construct
  source 1..20: mol_type = other RNA
catcctctgcttttgtcagt

SEQ ID NO: 6252 - RNA, 20 nt, synthetic construct
  source 1..20: mol_type = other RNA
aaagcagaggatggtggccc

SEQ ID NO: 6253 - RNA, 20 nt, synthetic construct
  source 1..20: mol_type = other RNA
gcagaggatggtggccctgg

SEQ ID NO: 6254 - RNA, 20 nt, synthetic construct
  source 1..20: mol_type = other RNA
gatggtggccctggaggcca

SEQ ID NO: 6255 - RNA, 20 nt, synthetic construct
  source 1..20: mol_type = other RNA
atggtggccctggaggccaa

SEQ ID NO: 6256 - RNA, 20 nt, synthetic construct
  source 1..20: mol_type = other RNA
gccctggaggccaagggaga

SEQ ID NO: 6257 - RNA, 20 nt, synthetic construct
  source 1..20: mol_type = other RNA
accttctcccttggcctcca

SEQ ID NO: 6258 - RNA, 20 nt, synthetic construct
  source 1..20: mol_type = other RNA
gaccttctcccttggcctcc

SEQ ID NO: 6259 - RNA, 20 nt, synthetic construct
  source 1..20: mol_type = other RNA
gtcaaagagaccttctccct

SEQ ID NO: 6260 - RNA, 20 nt, synthetic construct
  source 1..20: mol_type = other RNA
tgcatagggttagaaagcac

SEQ ID NO: 6261 - RNA, 20 nt, synthetic construct
  source 1..20: mol_type = other RNA
ttcttttatgggtctgcata

SEQ ID NO: 6262 - RNA, 20 nt, synthetic construct
  source 1..20: mol_type = other RNA
attcttttatgggtctgcat

SEQ ID NO: 6263 - RNA, 20 nt, synthetic construct
  source 1..20: mol_type = other RNA
cagacccataaaagaatccc

SEQ ID NO: 6264 - RNA, 20 nt, synthetic construct
  source 1..20: mol_type = other RNA
tgttcctgggattcttttat

SEQ ID NO: 6265 - RNA, 20 nt, synthetic construct
  source 1..20: mol_type = other RNA
aaagaatcccaggaacattt

SEQ ID NO: 6266 - RNA, 20 nt, synthetic construct
  source 1..20: mol_type = other RNA
agagattccaaaatgttcct

SEQ ID NO: 6267 - RNA, 20 nt, synthetic construct
  source 1..20: mol_type = other RNA
aagagattccaaaatgttcc

SEQ ID NO: 6268 - RNA, 20 nt, synthetic construct
  source 1..20: mol_type = other RNA
atcaagaatgttgatttcaa

SEQ ID NO: 6269 - RNA, 20 nt, synthetic construct
  source 1..20: mol_type = other RNA
tcaagaatgttgatttcaat

SEQ ID NO: 6270 - RNA, 20 nt, synthetic construct
  source 1..20: mol_type = other RNA
taacttgtccaaagctctgc

SEQ ID NO: 6271 - RNA, 20 nt, synthetic construct
  source 1..20: mol_type = other RNA
caaagctctgctggtttccc

SEQ ID NO: 6272 - RNA, 20 nt, synthetic construct
  source 1..20: mol_type = other RNA
ctgggaaaccagcagagctt

SEQ ID NO: 6273 - RNA, 20 nt, synthetic construct
  source 1..20: mol_type = other RNA
tgctggtttcccaggctgtc

SEQ ID NO: 6274 - RNA, 20 nt, synthetic construct
  source 1..20: mol_type = other RNA
gctggtttcccaggctgtct

SEQ ID NO: 6275 - RNA, 20 nt, synthetic construct
  source 1..20: mol_type = other RNA
cttggaggcccagacagcct

SEQ ID NO: 6276 - RNA, 20 nt, synthetic construct
  source 1..20: mol_type = other RNA
tcttggaggcccagacagcc

SEQ ID NO: 6277 - RNA, 20 nt, synthetic construct
  source 1..20: mol_type = other RNA
gtctgggcctccaagagatc

SEQ ID NO: 6278 - RNA, 20 nt, synthetic construct
  source 1..20: mol_type = other RNA
ctccaagagatcaggaccaa

SEQ ID NO: 6279 - RNA, 20 nt, synthetic construct
  source 1..20: mol_type = other RNA
ctttggtcctgatctcttgg

SEQ ID NO: 6280 - RNA, 20 nt, synthetic construct
  source 1..20: mol_type = other RNA
agcctttggtcctgatctct

SEQ ID NO: 6281 - RNA, 20 nt, synthetic construct
  source 1..20: mol_type = other RNA
accaaaggctcatcctgcat

SEQ ID NO: 6282 - RNA, 20 nt, synthetic construct
  source 1..20: mol_type = other RNA
tccaatgcaggatgagcctt

SEQ ID NO: 6283 - RNA, 20 nt, synthetic construct
  source 1..20: mol_type = other RNA
acttgtcacagttccaatgc

SEQ ID NO: 6284 - RNA, 20 nt, synthetic construct
  source 1..20: mol_type = other RNA
agctttgttctagaaaggtc

SEQ ID NO: 6285 - RNA, 20 nt, synthetic construct
  source 1..20: mol_type = other RNA
ttctagaacaaagctacacc

SEQ ID NO: 6286 - RNA, 20 nt, synthetic construct
  source 1..20: mol_type = other RNA
ggtgtagctttgttctagaa

SEQ ID NO: 6287 - RNA, 20 nt, synthetic construct
  source 1..20: mol_type = other RNA
caccaggaaagaagagtctt

SEQ ID NO: 6288 - RNA, 20 nt, synthetic construct
  source 1..20: mol_type = other RNA
ggaaagaagagtcttaggca

SEQ ID NO: 6289 - RNA, 20 nt, synthetic construct
  source 1..20: mol_type = other RNA
tgcctaagactcttctttcc

SEQ ID NO: 6290 - RNA, 20 nt, synthetic construct
  source 1..20: mol_type = other RNA
gcaaggaatcagatgtccta

SEQ ID NO: 6291 - RNA, 20 nt, synthetic construct
  source 1..20: mol_type = other RNA
aggtcatgtagagcagcctt

SEQ ID NO: 6292 - RNA, 20 nt, synthetic construct
  source 1..20: mol_type = other RNA
gctctacatgacctacatga

SEQ ID NO: 6293 - RNA, 20 nt, synthetic construct
  source 1..20: mol_type = other RNA
ctctacatgacctacatgat

SEQ ID NO: 6294 - RNA, 20 nt, synthetic construct
  source 1..20: mol_type = other RNA
ggaggtaacacccatcatgt

SEQ ID NO: 6295 - RNA, 20 nt, synthetic construct
  source 1..20: mol_type = other RNA
tgactgaatgggagatgagg

SEQ ID NO: 6296 - RNA, 20 nt, synthetic construct
  source 1..20: mol_type = other RNA
tctcccattcagtcaaccca

SEQ ID NO: 6297 - RNA, 20 nt, synthetic construct
  source 1..20: mol_type = other RNA
ctcccattcagtcaacccac

SEQ ID NO: 6298 - RNA, 20 nt, synthetic construct
  source 1..20: mol_type = other RNA
ttcagtcaacccacgggcac

SEQ ID NO: 6299 - RNA, 20 nt, synthetic construct
  source 1..20: mol_type = other RNA
tgcccgtgggttgactgaat

SEQ ID NO: 6300 - RNA, 20 nt, synthetic construct
  source 1..20: mol_type = other RNA
gtgcccgtgggttgactgaa

SEQ ID NO: 6301 - RNA, 20 nt, synthetic construct
  source 1..20: mol_type = other RNA
gcaggaagtccagtgcccgt

SEQ ID NO: 6302 - RNA, 20 nt, synthetic construct
  source 1..20: mol_type = other RNA
ggcaggaagtccagtgcccg

SEQ ID NO: 6303 - RNA, 20 nt, synthetic construct
  source 1..20: mol_type = other RNA
gagagggaagggtgtcgggc

SEQ ID NO: 6304 - RNA, 20 nt, synthetic construct
  source 1..20: mol_type = other RNA
tggggagagggaagggtgtc

SEQ ID NO: 6305 - RNA, 20 nt, synthetic construct
  source 1..20: mol_type = other RNA
atggggagagggaagggtgt

SEQ ID NO: 6306 - RNA, 20 nt, synthetic construct
  source 1..20: mol_type = other RNA
tccctctccccattcatgcc

SEQ ID NO: 6307 - RNA, 20 nt, synthetic construct
  source 1..20: mol_type = other RNA
gcatgaatggggagagggaa

SEQ ID NO: 6308 - RNA, 20 nt, synthetic construct
  source 1..20: mol_type = other RNA
ggcatgaatggggagaggga

SEQ ID NO: 6309 - RNA, 20 nt, synthetic construct
  source 1..20: mol_type = other RNA
tccaggcatgaatggggaga

SEQ ID NO: 6310 - RNA, 20 nt, synthetic construct
  source 1..20: mol_type = other RNA
ttccaggcatgaatggggag

SEQ ID NO: 6311 - RNA, 20 nt, synthetic construct
  source 1..20: mol_type = other RNA
aataattccaggcatgaatg

SEQ ID NO: 6312 - RNA, 20 nt, synthetic construct
  source 1..20: mol_type = other RNA
aaataattccaggcatgaat

SEQ ID NO: 6313 - RNA, 20 nt, synthetic construct
  source 1..20: mol_type = other RNA
aaaataattccaggcatgaa

SEQ ID NO: 6314 - RNA, 20 nt, synthetic construct
  source 1..20: mol_type = other RNA
tcattagtgaaaataattcc

SEQ ID NO: 6315 - RNA, 20 nt, synthetic construct
  source 1..20: mol_type = other RNA
ttattttcactaatgacacc

SEQ ID NO: 6316 - RNA, 20 nt, synthetic construct
  source 1..20: mol_type = other RNA
tattttcactaatgacacca

SEQ ID NO: 6317 - RNA, 20 nt, synthetic construct
  source 1..20: mol_type = other RNA
tgacaccagggattcactaa

SEQ ID NO: 6318 - RNA, 20 nt, synthetic construct
  source 1..20: mol_type = other RNA
agcatccattagtgaatccc

SEQ ID NO: 6319 - RNA, 20 nt, synthetic construct
  source 1..20: mol_type = other RNA
cctgtcctatttgtctccac

SEQ ID NO: 6320 - RNA, 20 nt, synthetic construct
  source 1..20: mol_type = other RNA
ccagtggagacaaataggac

SEQ ID NO: 6321 - RNA, 20 nt, synthetic construct
  source 1..20: mol_type = other RNA
cactgccagtggagacaaat

SEQ ID NO: 6322 - RNA, 20 nt, synthetic construct
  source 1..20: mol_type = other RNA
gggaagtcaaacactgccag

SEQ ID NO: 6323 - RNA, 20 nt, synthetic construct
  source 1..20: mol_type = other RNA
aagaaatggtcaacactaca

SEQ ID NO: 6324 - RNA, 20 nt, synthetic construct
  source 1..20: mol_type = other RNA
aaagaaatggtcaacactac

SEQ ID NO: 6325 - RNA, 20 nt, synthetic construct
  source 1..20: mol_type = other RNA
aagttctgggaggaaagaaa

SEQ ID NO: 6326 - RNA, 20 nt, synthetic construct
  source 1..20: mol_type = other RNA
ttcctcccagaacttctgcc

SEQ ID NO: 6327 - RNA, 20 nt, synthetic construct
  source 1..20: mol_type = other RNA
tcctcccagaacttctgcct

SEQ ID NO: 6328 - RNA, 20 nt, synthetic construct
  source 1..20: mol_type = other RNA
gcccaggcagaagttctggg

SEQ ID NO: 6329 - RNA, 20 nt, synthetic construct
  source 1..20: mol_type = other RNA
gcggcccaggcagaagttct

SEQ ID NO: 6330 - RNA, 20 nt, synthetic construct
  source 1..20: mol_type = other RNA
ggcggcccaggcagaagttc

SEQ ID NO: 6331 - RNA, 20 nt, synthetic construct
  source 1..20: mol_type = other RNA
gtatggagtcatggcggccc

SEQ ID NO: 6332 - RNA, 20 nt, synthetic construct
  source 1..20: mol_type = other RNA
gccatgactccatactctcc

SEQ ID NO: 6333 - RNA, 20 nt, synthetic construct
  source 1..20: mol_type = other RNA
aggagagtatggagtcatgg

SEQ ID NO: 6334 - RNA, 20 nt, synthetic construct
  source 1..20: mol_type = other RNA
accaggagagtatggagtca

SEQ ID NO: 6335 - RNA, 20 nt, synthetic construct
  source 1..20: mol_type = other RNA
atactctcctggtttttgtc

SEQ ID NO: 6336 - RNA, 20 nt, synthetic construct
  source 1..20: mol_type = other RNA
tgacaaaaaccaggagagta

SEQ ID NO: 6337 - RNA, 20 nt, synthetic construct
  source 1..20: mol_type = other RNA
gagaccgcctgacaaaaacc

SEQ ID NO: 6338 - RNA, 20 nt, synthetic construct
  source 1..20: mol_type = other RNA
tgtcaggcggtctctcacac

SEQ ID NO: 6339 - RNA, 20 nt, synthetic construct
  source 1..20: mol_type = other RNA
aggcggtctctcacactggc

SEQ ID NO: 6340 - RNA, 20 nt, synthetic construct
  source 1..20: mol_type = other RNA
actggcaggcttccattctt

SEQ ID NO: 6341 - RNA, 20 nt, synthetic construct
  source 1..20: mol_type = other RNA
cgaaaattaagaccaaagaa

SEQ ID NO: 6342 - RNA, 20 nt, synthetic construct
  source 1..20: mol_type = other RNA
ggagagtggagcttgcagga

SEQ ID NO: 6343 - RNA, 20 nt, synthetic construct
  source 1..20: mol_type = other RNA
cggagagtggagcttgcagg

SEQ ID NO: 6344 - RNA, 20 nt, synthetic construct
  source 1..20: mol_type = other RNA
aggcggagagtggagcttgc

SEQ ID NO: 6345 - RNA, 20 nt, synthetic construct
  source 1..20: mol_type = other RNA
aggaaccatgaggcggagag

SEQ ID NO: 6346 - RNA, 20 nt, synthetic construct
  source 1..20: mol_type = other RNA
ctcatggttcctgttctcca

SEQ ID NO: 6347 - RNA, 20 nt, synthetic construct
  source 1..20: mol_type = other RNA
ggagaacaggaaccatgagg

SEQ ID NO: 6348 - RNA, 20 nt, synthetic construct
  source 1..20: mol_type = other RNA
tggttcctgttctccatggg

SEQ ID NO: 6349 - RNA, 20 nt, synthetic construct
  source 1..20: mol_type = other RNA
agaggccacccatggagaac

SEQ ID NO: 6350 - RNA, 20 nt, synthetic construct
  source 1..20: mol_type = other RNA
agctgggaagaggccaccca

SEQ ID NO: 6351 - RNA, 20 nt, synthetic construct
  source 1..20: mol_type = other RNA
ggcctcttcccagctccaga

SEQ ID NO: 6352 - RNA, 20 nt, synthetic construct
  source 1..20: mol_type = other RNA
ttccatctggagctgggaag

SEQ ID NO: 6353 - RNA, 20 nt, synthetic construct
  source 1..20: mol_type = other RNA
ggcaagttccatctggagct

SEQ ID NO: 6354 - RNA, 20 nt, synthetic construct
  source 1..20: mol_type = other RNA
tggcaagttccatctggagc

SEQ ID NO: 6355 - RNA, 20 nt, synthetic construct
  source 1..20: mol_type = other RNA
tgggcttggcaagttccatc

SEQ ID NO: 6356 - RNA, 20 nt, synthetic construct
  source 1..20: mol_type = other RNA
tgatgctatggatgtgggct

SEQ ID NO: 6357 - RNA, 20 nt, synthetic construct
  source 1..20: mol_type = other RNA
atgtgtgatgctatggatgt

SEQ ID NO: 6358 - RNA, 20 nt, synthetic construct
  source 1..20: mol_type = other RNA
aatgtgtgatgctatggatg

SEQ ID NO: 6359 - RNA, 20 nt, synthetic construct
  source 1..20: mol_type = other RNA
agcagaaatgtgtgatgcta

SEQ ID NO: 6360 - RNA, 20 nt, synthetic construct
  source 1..20: mol_type = other RNA
acacatttctgctgttctcc

SEQ ID NO: 6361 - RNA, 20 nt, synthetic construct
  source 1..20: mol_type = other RNA
gaggtgctgggggatgttcc

SEQ ID NO: 6362 - RNA, 20 nt, synthetic construct
  source 1..20: mol_type = other RNA
agtctgacgggaggtgctgg

SEQ ID NO: 6363 - RNA, 20 nt, synthetic construct
  source 1..20: mol_type = other RNA
gagtctgacgggaggtgctg

SEQ ID NO: 6364 - RNA, 20 nt, synthetic construct
  source 1..20: mol_type = other RNA
cgagtctgacgggaggtgct

SEQ ID NO: 6365 - RNA, 20 nt, synthetic construct
  source 1..20: mol_type = other RNA
gcgagtctgacgggaggtgc

SEQ ID NO: 6366 - RNA, 20 nt, synthetic construct
  source 1..20: mol_type = other RNA
attgtggcgagtctgacggg

SEQ ID NO: 6367 - RNA, 20 nt, synthetic construct
  source 1..20: mol_type = other RNA
ttcattgtggcgagtctgac

SEQ ID NO: 6368 - RNA, 20 nt, synthetic construct
  source 1..20: mol_type = other RNA
tttcattgtggcgagtctga

SEQ ID NO: 6369 - RNA, 20 nt, synthetic construct
  source 1..20: mol_type = other RNA
gacagagcagggtttcattg

SEQ ID NO: 6370 - RNA, 20 nt, synthetic construct
  source 1..20: mol_type = other RNA
gtggggtagaggacagagca

SEQ ID NO: 6371 - RNA, 20 nt, synthetic construct
  source 1..20: mol_type = other RNA
agtggggtagaggacagagc

SEQ ID NO: 6372 - RNA, 20 nt, synthetic construct
  source 1..20: mol_type = other RNA
gtaagtaatgagtggggtag

SEQ ID NO: 6373 - RNA, 20 nt, synthetic construct
  source 1..20: mol_type = other RNA
cccactcattacttaccatg

SEQ ID NO: 6374 - RNA, 20 nt, synthetic construct
  source 1..20: mol_type = other RNA
cacatggtaagtaatgagtg

SEQ ID NO: 6375 - RNA, 20 nt, synthetic construct
  source 1..20: mol_type = other RNA
ccacatggtaagtaatgagt

SEQ ID NO: 6376 - RNA, 20 nt, synthetic construct
  source 1..20: mol_type = other RNA
gccacatggtaagtaatgag

SEQ ID NO: 6377 - RNA, 20 nt, synthetic construct
  source 1..20: mol_type = other RNA
gagggaattcacaggccaca

SEQ ID NO: 6378 - RNA, 20 nt, synthetic construct
  source 1..20: mol_type = other RNA
caaggcaggagggaattcac

SEQ ID NO: 6379 - RNA, 20 nt, synthetic construct
  source 1..20: mol_type = other RNA
caagctgggacaaggcagga

SEQ ID NO: 6380 - RNA, 20 nt, synthetic construct
  source 1..20: mol_type = other RNA
gcaagctgggacaaggcagg

SEQ ID NO: 6381 - RNA, 20 nt, synthetic construct
  source 1..20: mol_type = other RNA
cttgtcccagcttgctcctc

SEQ ID NO: 6382 - RNA, 20 nt, synthetic construct
  source 1..20: mol_type = other RNA
ctgaggagcaagctgggaca

SEQ ID NO: 6383 - RNA, 20 nt, synthetic construct
  source 1..20: mol_type = other RNA
agagacctgaggagcaagct

SEQ ID NO: 6384 - RNA, 20 nt, synthetic construct
  source 1..20: mol_type = other RNA
tagagacctgaggagcaagc

SEQ ID NO: 6385 - RNA, 20 nt, synthetic construct
  source 1..20: mol_type = other RNA
cagaagggggtagagacctg

SEQ ID NO: 6386 - RNA, 20 nt, synthetic construct
  source 1..20: mol_type = other RNA
aaggtggtaaactcagaagg

SEQ ID NO: 6387 - RNA, 20 nt, synthetic construct
  source 1..20: mol_type = other RNA
gaaggtggtaaactcagaag

SEQ ID NO: 6388 - RNA, 20 nt, synthetic construct
  source 1..20: mol_type = other RNA
agaaggtggtaaactcagaa

SEQ ID NO: 6389 - RNA, 20 nt, synthetic construct
  source 1..20: mol_type = other RNA
cagaaggtggtaaactcaga

SEQ ID NO: 6390 - RNA, 20 nt, synthetic construct
  source 1..20: mol_type = other RNA
caaagtgagagatcagaagg

SEQ ID NO: 6391 - RNA, 20 nt, synthetic construct
  source 1..20: mol_type = other RNA
aggcaaagtgagagatcaga

SEQ ID NO: 6392 - RNA, 20 nt, synthetic construct
  source 1..20: mol_type = other RNA
tcactttgcctctgctaatc

SEQ ID NO: 6393 - RNA, 20 nt, synthetic construct
  source 1..20: mol_type = other RNA
tctgctaatctggcttcttc

SEQ ID NO: 6394 - RNA, 20 nt, synthetic construct
  source 1..20: mol_type = other RNA
tgaagaagccagattagcag

SEQ ID NO: 6395 - RNA, 20 nt, synthetic construct
  source 1..20: mol_type = other RNA
tccattatcctcatccaaac

SEQ ID NO: 6396 - RNA, 20 nt, synthetic construct
  source 1..20: mol_type = other RNA
gtttggatgaggataatgga

SEQ ID NO: 6397 - RNA, 20 nt, synthetic construct
  source 1..20: mol_type = other RNA
tgtttggatgaggataatgg

SEQ ID NO: 6398 - RNA, 20 nt, synthetic construct
  source 1..20: mol_type = other RNA
gcctgtttggatgaggataa

SEQ ID NO: 6399 - RNA, 20 nt, synthetic construct
  source 1..20: mol_type = other RNA
aggacgggcctgtttggatg

SEQ ID NO: 6400 - RNA, 20 nt, synthetic construct
  source 1..20: mol_type = other RNA
aggataaggacgggcctgtt

SEQ ID NO: 6401 - RNA, 20 nt, synthetic construct
  source 1..20: mol_type = other RNA
gcccgtccttatcctgagaa

SEQ ID NO: 6402 - RNA, 20 nt, synthetic construct
  source 1..20: mol_type = other RNA
tccattctcaggataaggac

SEQ ID NO: 6403 - RNA, 20 nt, synthetic construct
  source 1..20: mol_type = other RNA
atccattctcaggataagga

SEQ ID NO: 6404 - RNA, 20 nt, synthetic construct
  source 1..20: mol_type = other RNA
aggtatccattctcaggata

SEQ ID NO: 6405 - RNA, 20 nt, synthetic construct
  source 1..20: mol_type = other RNA
gtttctaggtatccattctc

SEQ ID NO: 6406 - RNA, 20 nt, synthetic construct
  source 1..20: mol_type = other RNA
gactgggtggggaagtttct

SEQ ID NO: 6407 - RNA, 20 nt, synthetic construct
  source 1..20: mol_type = other RNA
gcttgggataggactgggtg

SEQ ID NO: 6408 - RNA, 20 nt, synthetic construct
  source 1..20: mol_type = other RNA
ggcttgggataggactgggt

SEQ ID NO: 6409 - RNA, 20 nt, synthetic construct
  source 1..20: mol_type = other RNA
gggcttgggataggactggg

SEQ ID NO: 6410 - RNA, 20 nt, synthetic construct
  source 1..20: mol_type = other RNA
ccagggcttgggataggact

SEQ ID NO: 6411 - RNA, 20 nt, synthetic construct
  source 1..20: mol_type = other RNA
cccagggcttgggataggac

SEQ ID NO: 6412 - RNA, 20 nt, synthetic construct
  source 1..20: mol_type = other RNA
aatttcccagggcttgggat

SEQ ID NO: 6413 - RNA, 20 nt, synthetic construct
  source 1..20: mol_type = other RNA
gggataatttcccagggctt

SEQ ID NO: 6414 - RNA, 20 nt, synthetic construct
  source 1..20: mol_type = other RNA
tgggataatttcccagggct

SEQ ID NO: 6415 - RNA, 20 nt, synthetic construct
  source 1..20: mol_type = other RNA
aatactgggataatttccca

SEQ ID NO: 6416 - RNA, 20 nt, synthetic construct
  source 1..20: mol_type = other RNA
caatactgggataatttccc

SEQ ID NO: 6417 - RNA, 20 nt, synthetic construct
  source 1..20: mol_type = other RNA
gacatgaggcagacaatact

SEQ ID NO: 6418 - RNA, 20 nt, synthetic construct
  source 1..20: mol_type = other RNA
ggacatgaggcagacaatac

SEQ ID NO: 6419 - RNA, 20 nt, synthetic construct
  source 1..20: mol_type = other RNA
tctgcctcatgtccctggca

SEQ ID NO: 6420 - RNA, 20 nt, synthetic construct
  source 1..20: mol_type = other RNA
ttctccttgccagggacatg

SEQ ID NO: 6421 - RNA, 20 nt, synthetic construct
  source 1..20: mol_type = other RNA
gaaacgttttctccttgcca

SEQ ID NO: 6422 - RNA, 20 nt, synthetic construct
  source 1..20: mol_type = other RNA
agaaacgttttctccttgcc

SEQ ID NO: 6423 - RNA, 20 nt, synthetic construct
  source 1..20: mol_type = other RNA
tcttatacccaaaccagaaa

SEQ ID NO: 6424 - RNA, 20 nt, synthetic construct
  source 1..20: mol_type = other RNA
cttatacccaaaccagaaat

SEQ ID NO: 6425 - RNA, 20 nt, synthetic construct
  source 1..20: mol_type = other RNA
ttatacccaaaccagaaatg

SEQ ID NO: 6426 - RNA, 20 nt, synthetic construct
  source 1..20: mol_type = other RNA
tacccaaaccagaaatgggg

SEQ ID NO: 6427 - RNA, 20 nt, synthetic construct
  source 1..20: mol_type = other RNA
agcctccccatttctggttt

SEQ ID NO: 6428 - RNA, 20 nt, synthetic construct
  source 1..20: mol_type = other RNA
aagcctccccatttctggtt

SEQ ID NO: 6429 - RNA, 20 nt, synthetic construct
  source 1..20: mol_type = other RNA
gtgggaagcctccccatttc

SEQ ID NO: 6430 - RNA, 20 nt, synthetic construct
  source 1..20: mol_type = other RNA
ttcagcaaagagaagaacgt

SEQ ID NO: 6431 - RNA, 20 nt, synthetic construct
  source 1..20: mol_type = other RNA
attcagcaaagagaagaacg

SEQ ID NO: 6432 - RNA, 20 nt, synthetic construct
  source 1..20: mol_type = other RNA
gggcagggcttggtgatgga

SEQ ID NO: 6433 - RNA, 20 nt, synthetic construct
  source 1..20: mol_type = other RNA
gaatgggcagggcttggtga

SEQ ID NO: 6434 - RNA, 20 nt, synthetic construct
  source 1..20: mol_type = other RNA
gaggtagaatgggcagggct

SEQ ID NO: 6435 - RNA, 20 nt, synthetic construct
  source 1..20: mol_type = other RNA
ctgaagaggtagaatgggca

SEQ ID NO: 6436 - RNA, 20 nt, synthetic construct
  source 1..20: mol_type = other RNA
actgaagaggtagaatgggc

SEQ ID NO: 6437 - RNA, 20 nt, synthetic construct
  source 1..20: mol_type = other RNA
agtgactgaagaggtagaat

SEQ ID NO: 6438 - RNA, 20 nt, synthetic construct
  source 1..20: mol_type = other RNA
gagtgactgaagaggtagaa

SEQ ID NO: 6439 - RNA, 20 nt, synthetic construct
  source 1..20: mol_type = other RNA
gatctgaggagtgactgaag

SEQ ID NO: 6440 - RNA, 20 nt, synthetic construct
  source 1..20: mol_type = other RNA
cggacgggaagaaggatctg

SEQ ID NO: 6441 - RNA, 20 nt, synthetic construct
  source 1..20: mol_type = other RNA
tggagatgcggacgggaaga

SEQ ID NO: 6442 - RNA, 20 nt, synthetic construct
  source 1..20: mol_type = other RNA
gtggctgtggagatgcggac

SEQ ID NO: 6443 - RNA, 20 nt, synthetic construct
  source 1..20: mol_type = other RNA
tgtggctgtggagatgcgga

SEQ ID NO: 6444 - RNA, 20 nt, synthetic construct
  source 1..20: mol_type = other RNA
agggtgtggctgtggagatg

SEQ ID NO: 6445 - RNA, 20 nt, synthetic construct
  source 1..20: mol_type = other RNA
atggagggagggtgtggctg

SEQ ID NO: 6446 - RNA, 20 nt, synthetic construct
  source 1..20: mol_type = other RNA
gaggcaatggagggagggtg

SEQ ID NO: 6447 - RNA, 20 nt, synthetic construct
  source 1..20: mol_type = other RNA
gatgagaggcaatggaggga

SEQ ID NO: 6448 - RNA, 20 nt, synthetic construct
  source 1..20: mol_type = other RNA
tgatgagaggcaatggaggg

SEQ ID NO: 6449 - RNA, 20 nt, synthetic construct
  source 1..20: mol_type = other RNA
cagtgatgagaggcaatgga

SEQ ID NO: 6450 - RNA, 20 nt, synthetic construct
  source 1..20: mol_type = other RNA
gcagtgatgagaggcaatgg

SEQ ID NO: 6451 - RNA, 20 nt, synthetic construct
  source 1..20: mol_type = other RNA
agggcagtgatgagaggcaa

SEQ ID NO: 6452 - RNA, 20 nt, synthetic construct
  source 1..20: mol_type = other RNA
gggattagggcagtgatgag

SEQ ID NO: 6453 - RNA, 20 nt, synthetic construct
  source 1..20: mol_type = other RNA
atcactgccctaatccccaa

SEQ ID NO: 6454 - RNA, 20 nt, synthetic construct
  source 1..20: mol_type = other RNA
tcactgccctaatccccaag

SEQ ID NO: 6455 - RNA, 20 nt, synthetic construct
  source 1..20: mol_type = other RNA
cacgtaccccttggggatta

SEQ ID NO: 6456 - RNA, 20 nt, synthetic construct
  source 1..20: mol_type = other RNA
gcacgtaccccttggggatt

SEQ ID NO: 6457 - RNA, 20 nt, synthetic construct
  source 1..20: mol_type = other RNA
ctgggtgcacgtaccccttg

SEQ ID NO: 6458 - RNA, 20 nt, synthetic construct
  source 1..20: mol_type = other RNA
cctgggtgcacgtacccctt

SEQ ID NO: 6459 - RNA, 20 nt, synthetic construct
  source 1..20: mol_type = other RNA
ccctgggtgcacgtacccct

SEQ ID NO: 6460 - RNA, 20 nt, synthetic construct
  source 1..20: mol_type = other RNA
aggatttttagagtgctgtt

SEQ ID NO: 6461 - RNA, 20 nt, synthetic construct
  source 1..20: mol_type = other RNA
taggatttttagagtgctgt

SEQ ID NO: 6462 - RNA, 20 nt, synthetic construct
  source 1..20: mol_type = other RNA
actctaaaaatcctaaacat

SEQ ID NO: 6463 - RNA, 20 nt, synthetic construct
  source 1..20: mol_type = other RNA
ataacatagcaccaatgttt

SEQ ID NO: 6464 - RNA, 20 nt, synthetic construct
  source 1..20: mol_type = other RNA
tgtctagatccaagtatttc

SEQ ID NO: 6465 - RNA, 20 nt, synthetic construct
  source 1..20: mol_type = other RNA
aaagctcatccagaaatact

SEQ ID NO: 6466 - RNA, 20 nt, synthetic construct
  source 1..20: mol_type = other RNA
gagctttcctattttaaaaa

SEQ ID NO: 6467 - RNA, 20 nt, synthetic construct
  source 1..20: mol_type = other RNA
agctttcctattttaaaaat

SEQ ID NO: 6468 - RNA, 20 nt, synthetic construct
  source 1..20: mol_type = other RNA
tttttacccatttttaaaat

SEQ ID NO: 6469 - RNA, 20 nt, synthetic construct
  source 1..20: mol_type = other RNA
agtccctgattcagcttttc

SEQ ID NO: 6470 - RNA, 20 nt, synthetic construct
  source 1..20: mol_type = other RNA
aaaagctgaatcagggactt

SEQ ID NO: 6471 - RNA, 20 nt, synthetic construct
  source 1..20: mol_type = other RNA
gaaaagctgaatcagggact

SEQ ID NO: 6472 - RNA, 20 nt, synthetic construct
  source 1..20: mol_type = other RNA
tagcctgaaaagctgaatca

SEQ ID NO: 6473 - RNA, 20 nt, synthetic construct
  source 1..20: mol_type = other RNA
gtagcctgaaaagctgaatc

SEQ ID NO: 6474 - RNA, 20 nt, synthetic construct
  source 1..20: mol_type = other RNA
tcaggctacatcaatacccc

SEQ ID NO: 6475 - RNA, 20 nt, synthetic construct
  source 1..20: mol_type = other RNA
catttgtgttgaagcaccag

SEQ ID NO: 6476 - RNA, 20 nt, synthetic construct
  source 1..20: mol_type = other RNA
gcatttgtgttgaagcacca

SEQ ID NO: 6477 - RNA, 20 nt, synthetic construct
  source 1..20: mol_type = other RNA
agcatttgtgttgaagcacc

SEQ ID NO: 6478 - RNA, 20 nt, synthetic construct
  source 1..20: mol_type = other RNA
atgctgacccttgtactgac

SEQ ID NO: 6479 - RNA, 20 nt, synthetic construct
  source 1..20: mol_type = other RNA
ctaattgccagtcagtacaa

SEQ ID NO: 6480 - RNA, 20 nt, synthetic construct
  source 1..20: mol_type = other RNA
actaattgccagtcagtaca

SEQ ID NO: 6481 - RNA, 20 nt, synthetic construct
  source 1..20: mol_type = other RNA
tgatctgagggttgaattca

SEQ ID NO: 6482 - RNA, 20 nt, synthetic construct
  source 1..20: mol_type = other RNA
ttgatctgagggttgaattc

SEQ ID NO: 6483 - RNA, 20 nt, synthetic construct
  source 1..20: mol_type = other RNA
cagatcaatgtctataaaat

SEQ ID NO: 6484 - RNA, 20 nt, synthetic construct
  source 1..20: mol_type = other RNA
ttttatagacattgatctga

SEQ ID NO: 6485 - RNA, 20 nt, synthetic construct
  source 1..20: mol_type = other RNA
attttatagacattgatctg

SEQ ID NO: 6486 - RNA, 20 nt, synthetic construct
  source 1..20: mol_type = other RNA
tctataaaattggctgtaag

SEQ ID NO: 6487 - RNA, 20 nt, synthetic construct
  source 1..20: mol_type = other RNA
ataaaattggctgtaagagg

SEQ ID NO: 6488 - RNA, 20 nt, synthetic construct
  source 1..20: mol_type = other RNA
ctcacagtaatgggaatcaa

SEQ ID NO: 6489 - RNA, 20 nt, synthetic construct
  source 1..20: mol_type = other RNA
actcacagtaatgggaatca

SEQ ID NO: 6490 - RNA, 20 nt, synthetic construct
  source 1..20: mol_type = other RNA
cagctcttactcacagtaat

SEQ ID NO: 6491 - RNA, 20 nt, synthetic construct
  source 1..20: mol_type = other RNA
acagctcttactcacagtaa

SEQ ID NO: 6492 - RNA, 20 nt, synthetic construct
  source 1..20: mol_type = other RNA
tgttggctgcaaggggattt

SEQ ID NO: 6493 - RNA, 20 nt, synthetic construct
  source 1..20: mol_type = other RNA
aattttgtgttggctgcaag

SEQ ID NO: 6494 - RNA, 20 nt, synthetic construct
  source 1..20: mol_type = other RNA
aaattttgtgttggctgcaa

SEQ ID NO: 6495 - RNA, 20 nt, synthetic construct
  source 1..20: mol_type = other RNA
taaattttgtgttggctgca

SEQ ID NO: 6496 - RNA, 20 nt, synthetic construct
  source 1..20: mol_type = other RNA
gcagggggtaaattttgtgt

SEQ ID NO: 6497 - RNA, 20 nt, synthetic construct
  source 1..20: mol_type = other RNA
aaatttaccccctgctgcct

SEQ ID NO: 6498 - RNA, 20 nt, synthetic construct
  source 1..20: mol_type = other RNA
tggcactccgaggcagcagg

SEQ ID NO: 6499 - RNA, 20 nt, synthetic construct
  source 1..20: mol_type = other RNA
ttggcactccgaggcagcag

SEQ ID NO: 6500 - RNA, 20 nt, synthetic construct
  source 1..20: mol_type = other RNA
attggcactccgaggcagca

SEQ ID NO: 6501 - RNA, 20 nt, synthetic construct
  source 1..20: mol_type = other RNA
aattggcactccgaggcagc

SEQ ID NO: 6502 - RNA, 20 nt, synthetic construct
  source 1..20: mol_type = other RNA
ttattttaattggcactccg

SEQ ID NO: 6503 - RNA, 20 nt, synthetic construct
  source 1..20: mol_type = other RNA
ttggtttttattattttaat

SEQ ID NO: 6504 - RNA, 20 nt, synthetic construct
  source 1..20: mol_type = other RNA
aataataaaaaccaaaaccg

SEQ ID NO: 6505 - RNA, 20 nt, synthetic construct
  source 1..20: mol_type = other RNA
ataataaaaaccaaaaccgt

SEQ ID NO: 6506 - RNA, 20 nt, synthetic construct
  source 1..20: mol_type = other RNA
attacatctgcccacggttt

SEQ ID NO: 6507 - RNA, 20 nt, synthetic construct
  source 1..20: mol_type = other RNA
aaactaattacatctgccca

SEQ ID NO: 6508 - RNA, 20 nt, synthetic construct
  source 1..20: mol_type = other RNA
agatgtaattagtttgagaa

SEQ ID NO: 6509 - RNA, 20 nt, synthetic construct
  source 1..20: mol_type = other RNA
taacttgtttgcttggcatg

SEQ ID NO: 6510 - RNA, 20 nt, synthetic construct
  source 1..20: mol_type = other RNA
agcaaacaagttaacccctt

SEQ ID NO: 6511 - RNA, 20 nt, synthetic construct
  source 1..20: mol_type = other RNA
aaggggttaacttgtttgct

SEQ ID NO: 6512 - RNA, 20 nt, synthetic construct
  source 1..20: mol_type = other RNA
ttctgtatatgtcaccaaag

SEQ ID NO: 6513 - RNA, 20 nt, synthetic construct
  source 1..20: mol_type = other RNA
attctgtatatgtcaccaaa

SEQ ID NO: 6514 - RNA, 20 nt, synthetic construct
  source 1..20: mol_type = other RNA
tattctgtatatgtcaccaa

SEQ ID NO: 6515 - RNA, 20 nt, synthetic construct
  source 1..20: mol_type = other RNA
gtgacatatacagaataatc

SEQ ID NO: 6516 - RNA, 20 nt, synthetic construct
  source 1..20: mol_type = other RNA
atacagaataatctggacaa

SEQ ID NO: 6517 - RNA, 20 nt, synthetic construct
  source 1..20: mol_type = other RNA
tacagaataatctggacaaa

SEQ ID NO: 6518 - RNA, 20 nt, synthetic construct
  source 1..20: mol_type = other RNA
catttcttgtgctatttgcc

SEQ ID NO: 6519 - RNA, 20 nt, synthetic construct
  source 1..20: mol_type = other RNA
ttttcaatattacaacttcc

SEQ ID NO: 6520 - RNA, 20 nt, synthetic construct
  source 1..20: mol_type = other RNA
aaactgtgctcttctgagaa

SEQ ID NO: 6521 - RNA, 20 nt, synthetic construct
  source 1..20: mol_type = other RNA
aactgtgctcttctgagaat

SEQ ID NO: 6522 - RNA, 20 nt, synthetic construct
  source 1..20: mol_type = other RNA
cttctgagaatgggaaaatg

SEQ ID NO: 6523 - RNA, 20 nt, synthetic construct
  source 1..20: mol_type = other RNA
gaaaatgaggacataaactc

SEQ ID NO: 6524 - RNA, 20 nt, synthetic construct
  source 1..20: mol_type = other RNA
acataaactctggttccaaa

SEQ ID NO: 6525 - RNA, 20 nt, synthetic construct
  source 1..20: mol_type = other RNA
aaactctggttccaaatggt

SEQ ID NO: 6526 - RNA, 20 nt, synthetic construct
  source 1..20: mol_type = other RNA
aaactgcacttccaaccatt

SEQ ID NO: 6527 - RNA, 20 nt, synthetic construct
  source 1..20: mol_type = other RNA
ggttggaagtgcagtttatg

SEQ ID NO: 6528 - RNA, 20 nt, synthetic construct
  source 1..20: mol_type = other RNA
gaagtgcagtttatgtggtc

SEQ ID NO: 6529 - RNA, 20 nt, synthetic construct
  source 1..20: mol_type = other RNA
gaaagtttttttaatgaaag

SEQ ID NO: 6530 - RNA, 20 nt, synthetic construct
  source 1..20: mol_type = other RNA
tgaaagtttttttaatgaaa

SEQ ID NO: 6531 - RNA, 20 nt, synthetic construct
  source 1..20: mol_type = other RNA
ttgaaagtttttttaatgaa

SEQ ID NO: 6532 - RNA, 20 nt, synthetic construct
  source 1..20: mol_type = other RNA
tttcaagattccacttgatc

SEQ ID NO: 6533 - RNA, 20 nt, synthetic construct
  source 1..20: mol_type = other RNA
ttcaagattccacttgatcc

SEQ ID NO: 6534 - RNA, 20 nt, synthetic construct
  source 1..20: mol_type = other RNA
tcgaagaaacccggatcaag

SEQ ID NO: 6535 - RNA, 20 nt, synthetic construct
  source 1..20: mol_type = other RNA
aatacattttcgaagaaacc

SEQ ID NO: 6536 - RNA, 20 nt, synthetic construct
  source 1..20: mol_type = other RNA
tttacaaatataattcttat

SEQ ID NO: 6537 - RNA, 20 nt, synthetic construct
  source 1..20: mol_type = other RNA
ttacaaatataattcttata

SEQ ID NO: 6538 - RNA, 20 nt, synthetic construct
  source 1..20: mol_type = other RNA
acagacttcagctgtgtagc

SEQ ID NO: 6539 - RNA, 20 nt, synthetic construct
  source 1..20: mol_type = other RNA
gaacgttcttgaaagactgc

SEQ ID NO: 6540 - RNA, 20 nt, synthetic construct
  source 1..20: mol_type = other RNA
aacgttcttgaaagactgct

SEQ ID NO: 6541 - RNA, 20 nt, synthetic construct
  source 1..20: mol_type = other RNA
gcttgatactctttcagagg

SEQ ID NO: 6542 - RNA, 20 nt, synthetic construct
  source 1..20: mol_type = other RNA
tgaaagagtatcaagctcag

SEQ ID NO: 6543 - RNA, 20 nt, synthetic construct
  source 1..20: mol_type = other RNA
tgagcttgatactctttcag

SEQ ID NO: 6544 - RNA, 20 nt, synthetic construct
  source 1..20: mol_type = other RNA
agagtatcaagctcagtggt

SEQ ID NO: 6545 - RNA, 20 nt, synthetic construct
  source 1..20: mol_type = other RNA
gttcctgtcccacccatctc

SEQ ID NO: 6546 - RNA, 20 nt, synthetic construct
  source 1..20: mol_type = other RNA
ttcctgtcccacccatctct

SEQ ID NO: 6547 - RNA, 20 nt, synthetic construct
  source 1..20: mol_type = other RNA
tcccacccatctctgggatg

SEQ ID NO: 6548 - RNA, 20 nt, synthetic construct
  source 1..20: mol_type = other RNA
atcccagagatgggtgggac

SEQ ID NO: 6549 - RNA, 20 nt, synthetic construct
  source 1..20: mol_type = other RNA
tcctcatcccagagatgggt

SEQ ID NO: 6550 - RNA, 20 nt, synthetic construct
  source 1..20: mol_type = other RNA
ctcctcatcccagagatggg

SEQ ID NO: 6551 - RNA, 20 nt, synthetic construct
  source 1..20: mol_type = other RNA
gaactcctcatcccagagat

SEQ ID NO: 6552 - RNA, 20 nt, synthetic construct
  source 1..20: mol_type = other RNA
agaactcctcatcccagaga

SEQ ID NO: 6553 - RNA, 20 nt, synthetic construct
  source 1..20: mol_type = other RNA
ctgggatgaggagttctcca

SEQ ID NO: 6554 - RNA, 20 nt, synthetic construct
  source 1..20: mol_type = other RNA
ctccatggtgaccctgagtc

SEQ ID NO: 6555 - RNA, 20 nt, synthetic construct
  source 1..20: mol_type = other RNA
agcctgactcagggtcacca

SEQ ID NO: 6556 - RNA, 20 nt, synthetic construct
  source 1..20: mol_type = other RNA
tgcagaagaagcctgactca

SEQ ID NO: 6557 - RNA, 20 nt, synthetic construct
  source 1..20: mol_type = other RNA
gtgcagaagaagcctgactc

SEQ ID NO: 6558 - RNA, 20 nt, synthetic construct
  source 1..20: mol_type = other RNA
ttcttctgcacccctctgcc

SEQ ID NO: 6559 - RNA, 20 nt, synthetic construct
  source 1..20: mol_type = other RNA
acccctctgcctggttaatg

SEQ ID NO: 6560 - RNA, 20 nt, synthetic construct
  source 1..20: mol_type = other RNA
tcctcattaaccaggcagag

SEQ ID NO: 6561 - RNA, 20 nt, synthetic construct
  source 1..20: mol_type = other RNA
gtcctcattaaccaggcaga

SEQ ID NO: 6562 - RNA, 20 nt, synthetic construct
  source 1..20: mol_type = other RNA
agtcctcattaaccaggcag

SEQ ID NO: 6563 - RNA, 20 nt, synthetic construct
  source 1..20: mol_type = other RNA
cagttgagtcctcattaacc

SEQ ID NO: 6564 - RNA, 20 nt, synthetic construct
  source 1..20: mol_type = other RNA
gaaagggtttgtttgcagat

SEQ ID NO: 6565 - RNA, 20 nt, synthetic construct
  source 1..20: mol_type = other RNA
agaaagggtttgtttgcaga

SEQ ID NO: 6566 - RNA, 20 nt, synthetic construct
  source 1..20: mol_type = other RNA
tagagagaaaaatgcagaaa

SEQ ID NO: 6567 - RNA, 20 nt, synthetic construct
  source 1..20: mol_type = other RNA
ctagagagaaaaatgcagaa

SEQ ID NO: 6568 - RNA, 20 nt, synthetic construct
  source 1..20: mol_type = other RNA
cacgagtgagttatgtcaga

SEQ ID NO: 6569 - RNA, 20 nt, synthetic construct
  source 1..20: mol_type = other RNA
agttatgtcagatggtataa

SEQ ID NO: 6570 - RNA, 20 nt, synthetic construct
  source 1..20: mol_type = other RNA
gttatgtcagatggtataat

SEQ ID NO: 6571 - RNA, 20 nt, synthetic construct
  source 1..20: mol_type = other RNA
gtataatgggaaaaagacaa

SEQ ID NO: 6572 - RNA, 20 nt, synthetic construct
  source 1..20: mol_type = other RNA
acaaaggatatttgaatcta

SEQ ID NO: 6573 - RNA, 20 nt, synthetic construct
  source 1..20: mol_type = other RNA
gatatttgaatctaaggaca

SEQ ID NO: 6574 - RNA, 20 nt, synthetic construct
  source 1..20: mol_type = other RNA
atatttgaatctaaggacat

SEQ ID NO: 6575 - RNA, 20 nt, synthetic construct
  source 1..20: mol_type = other RNA
ttgaatctaaggacatgggc

SEQ ID NO: 6576 - RNA, 20 nt, synthetic construct
  source 1..20: mol_type = other RNA
ctaaggacatgggctggatc

SEQ ID NO: 6577 - RNA, 20 nt, synthetic construct
  source 1..20: mol_type = other RNA
acatgggctggatcaggtga

SEQ ID NO: 6578 - RNA, 20 nt, synthetic construct
  source 1..20: mol_type = other RNA
catgggctggatcaggtgaa

SEQ ID NO: 6579 - RNA, 20 nt, synthetic construct
  source 1..20: mol_type = other RNA
ggctggatcaggtgaaggga

SEQ ID NO: 6580 - RNA, 20 nt, synthetic construct
  source 1..20: mol_type = other RNA
ctgtttctgcttctttagtt

SEQ ID NO: 6581 - RNA, 20 nt, synthetic construct
  source 1..20: mol_type = other RNA
tgtttctgcttctttagttt

SEQ ID NO: 6582 - RNA, 20 nt, synthetic construct
  source 1..20: mol_type = other RNA
gtttctgcttctttagtttg

SEQ ID NO: 6583 - RNA, 20 nt, synthetic construct
  source 1..20: mol_type = other RNA
tctgcttctttagtttgggg

SEQ ID NO: 6584 - RNA, 20 nt, synthetic construct
  source 1..20: mol_type = other RNA
gcttctttagtttggggagg

SEQ ID NO: 6585 - RNA, 20 nt, synthetic construct
  source 1..20: mol_type = other RNA
ttagtttggggaggaggata

SEQ ID NO: 6586 - RNA, 20 nt, synthetic construct
  source 1..20: mol_type = other RNA
tggggaggaggataaggaaa

SEQ ID NO: 6587 - RNA, 20 nt, synthetic construct
  source 1..20: mol_type = other RNA
ggggaggaggataaggaaaa

SEQ ID NO: 6588 - RNA, 20 nt, synthetic construct
  source 1..20: mol_type = other RNA
aggaggataaggaaaagggt

SEQ ID NO: 6589 - RNA, 20 nt, synthetic construct
  source 1..20: mol_type = other RNA
acaaacttaccctcccacat

SEQ ID NO: 6590 - RNA, 20 nt, synthetic construct
  source 1..20: mol_type = other RNA
caaacttaccctcccacata

SEQ ID NO: 6591 - RNA, 20 nt, synthetic construct
  source 1..20: mol_type = other RNA
aaacttaccctcccacatag

SEQ ID NO: 6592 - RNA, 20 nt, synthetic construct
  source 1..20: mol_type = other RNA
gaagcatcccctatgtggga

SEQ ID NO: 6593 - RNA, 20 nt, synthetic construct
  source 1..20: mol_type = other RNA
tgaagcatcccctatgtggg

SEQ ID NO: 6594 - RNA, 20 nt, synthetic construct
  source 1..20: mol_type = other RNA
acatgaagcatcccctatgt

SEQ ID NO: 6595 - RNA, 20 nt, synthetic construct
  source 1..20: mol_type = other RNA
gacatgaagcatcccctatg

SEQ ID NO: 6596 - RNA, 20 nt, synthetic construct
  source 1..20: mol_type = other RNA
gatgcttcatgtcaagccac

SEQ ID NO: 6597 - RNA, 20 nt, synthetic construct
  source 1..20: mol_type = other RNA
agacggaggcattagaccag

SEQ ID NO: 6598 - RNA, 20 nt, synthetic construct
  source 1..20: mol_type = other RNA
ttttgaactaaagaagacgg

SEQ ID NO: 6599 - RNA, 20 nt, synthetic construct
  source 1..20: mol_type = other RNA
taattttgaactaaagaaga

SEQ ID NO: 6600 - RNA, 20 nt, synthetic construct
  source 1..20: mol_type = other RNA
ggaatcatgtttgcaatatt

SEQ ID NO: 6601 - RNA, 20 nt, synthetic construct
  source 1..20: mol_type = other RNA
caaacatgattccaccatgt

SEQ ID NO: 6602 - RNA, 20 nt, synthetic construct
  source 1..20: mol_type = other RNA
cacaactgaaaccaacatgg

SEQ ID NO: 6603 - RNA, 20 nt, synthetic construct
  source 1..20: mol_type = other RNA
gcacacaactgaaaccaaca

SEQ ID NO: 6604 - RNA, 20 nt, synthetic construct
  source 1..20: mol_type = other RNA
tccctgactgcacacaagtc

SEQ ID NO: 6605 - RNA, 20 nt, synthetic construct
  source 1..20: mol_type = other RNA
ccctgactgcacacaagtca

SEQ ID NO: 6606 - RNA, 20 nt, synthetic construct
  source 1..20: mol_type = other RNA
ccctgacttgtgtgcagtca

SEQ ID NO: 6607 - RNA, 20 nt, synthetic construct
  source 1..20: mol_type = other RNA
tccctgacttgtgtgcagtc

SEQ ID NO: 6608 - RNA, 20 nt, synthetic construct
  source 1..20: mol_type = other RNA
ctaaagaatgacaagcaaag

SEQ ID NO: 6609 - RNA, 20 nt, synthetic construct
  source 1..20: mol_type = other RNA
gacaagcaaagcggcatccc

SEQ ID NO: 6610 - RNA, 20 nt, synthetic construct
  source 1..20: mol_type = other RNA
acaagcaaagcggcatccca

SEQ ID NO: 6611 - RNA, 20 nt, synthetic construct
  source 1..20: mol_type = other RNA
aagcggcatcccagggctac

SEQ ID NO: 6612 - RNA, 20 nt, synthetic construct
  source 1..20: mol_type = other RNA
cccagggctactggttgaac

SEQ ID NO: 6613 - RNA, 20 nt, synthetic construct
  source 1..20: mol_type = other RNA
cctgttcaaccagtagccct

SEQ ID NO: 6614 - RNA, 20 nt, synthetic construct
  source 1..20: mol_type = other RNA
tcctgttcaaccagtagccc

SEQ ID NO: 6615 - RNA, 20 nt, synthetic construct
  source 1..20: mol_type = other RNA
ctggttgaacaggaaccctg

SEQ ID NO: 6616 - RNA, 20 nt, synthetic construct
  source 1..20: mol_type = other RNA
aggtcatctcaatggccaca

SEQ ID NO: 6617 - RNA, 20 nt, synthetic construct
  source 1..20: mol_type = other RNA
aaggtcatctcaatggccac

SEQ ID NO: 6618 - RNA, 20 nt, synthetic construct
  source 1..20: mol_type = other RNA
gcttgagaaggtcatctcaa

SEQ ID NO: 6619 - RNA, 20 nt, synthetic construct
  source 1..20: mol_type = other RNA
gctcaacaggaagcttgaga

SEQ ID NO: 6620 - RNA, 20 nt, synthetic construct
  source 1..20: mol_type = other RNA
gcttcctgttgagccttcac

SEQ ID NO: 6621 - RNA, 20 nt, synthetic construct
  source 1..20: mol_type = other RNA
cttcctgttgagccttcact

SEQ ID NO: 6622 - RNA, 20 nt, synthetic construct
  source 1..20: mol_type = other RNA
ttgagccttcactgggacac

SEQ ID NO: 6623 - RNA, 20 nt, synthetic construct
  source 1..20: mol_type = other RNA
tgagccttcactgggacact

SEQ ID NO: 6624 - RNA, 20 nt, synthetic construct
  source 1..20: mol_type = other RNA
cgctcccagtgtcccagtga

SEQ ID NO: 6625 - RNA, 20 nt, synthetic construct
  source 1..20: mol_type = other RNA
tgtgcgtatgtgtatgtatc

SEQ ID NO: 6626 - RNA, 20 nt, synthetic construct
  source 1..20: mol_type = other RNA
atgaagtctgacatttttca

SEQ ID NO: 6627 - RNA, 20 nt, synthetic construct
  source 1..20: mol_type = other RNA
gacttcatactgataatctg

SEQ ID NO: 6628 - RNA, 20 nt, synthetic construct
  source 1..20: mol_type = other RNA
acttcatactgataatctgt

SEQ ID NO: 6629 - RNA, 20 nt, synthetic construct
  source 1..20: mol_type = other RNA
caatctttttgtttcataaa

SEQ ID NO: 6630 - RNA, 20 nt, synthetic construct
  source 1..20: mol_type = other RNA
tgcttttcgagattataaac

SEQ ID NO: 6631 - RNA, 20 nt, synthetic construct
  source 1..20: mol_type = other RNA
gcttttcgagattataaact

SEQ ID NO: 6632 - RNA, 20 nt, synthetic construct
  source 1..20: mol_type = other RNA
tacgttcaagtcagttgttc

SEQ ID NO: 6633 - RNA, 20 nt, synthetic construct
  source 1..20: mol_type = other RNA
gtaaaaatattcacagaaat

SEQ ID NO: 6634 - RNA, 20 nt, synthetic construct
  source 1..20: mol_type = other RNA
tttctgtgaatatttttaca

SEQ ID NO: 6635 - RNA, 20 nt, synthetic construct
  source 1..20: mol_type = other RNA
aaaatattcacagaaattgg

SEQ ID NO: 6636 - RNA, 20 nt, synthetic construct
  source 1..20: mol_type = other RNA
taacatttgcaaccttagaa

SEQ ID NO: 6637 - RNA, 20 nt, synthetic construct
  source 1..20: mol_type = other RNA
taaacatgtctgcctttcta

SEQ ID NO: 6638 - RNA, 20 nt, synthetic construct
  source 1..20: mol_type = other RNA
ttggaatttataaacggact

SEQ ID NO: 6639 - RNA, 20 nt, synthetic construct
  source 1..20: mol_type = other RNA
ttataaattccaatttcaca

SEQ ID NO: 6640 - RNA, 20 nt, synthetic construct
  source 1..20: mol_type = other RNA
gtgaaattggaatttataaa

SEQ ID NO: 6641 - RNA, 20 nt, synthetic construct
  source 1..20: mol_type = other RNA
gtttttaatccatgtgaaat

SEQ ID NO: 6642 - RNA, 20 nt, synthetic construct
  source 1..20: mol_type = other RNA
aatatcctgtacatgcatta

SEQ ID NO: 6643 - RNA, 20 nt, synthetic construct
  source 1..20: mol_type = other RNA
tcctgtacatgcattaaggc

SEQ ID NO: 6644 - RNA, 20 nt, synthetic construct
  source 1..20: mol_type = other RNA
accagccttaatgcatgtac

SEQ ID NO: 6645 - RNA, 20 nt, synthetic construct
  source 1..20: mol_type = other RNA
tggtgactgctaaagtctct

SEQ ID NO: 6646 - RNA, 20 nt, synthetic construct
  source 1..20: mol_type = other RNA
ggtgactgctaaagtctctt

SEQ ID NO: 6647 - RNA, 20 nt, synthetic construct
  source 1..20: mol_type = other RNA
tctcttgggaatctacaaat

SEQ ID NO: 6648 - RNA, 20 nt, synthetic construct
  source 1..20: mol_type = other RNA
ggaaatcacacgcagattac

SEQ ID NO: 6649 - RNA, 20 nt, synthetic construct
  source 1..20: mol_type = other RNA
gaaatcacacgcagattact

SEQ ID NO: 6650 - RNA, 20 nt, synthetic construct
  source 1..20: mol_type = other RNA
atcttgcttttttttttttt

SEQ ID NO: 6651 - RNA, 20 nt, synthetic construct
  source 1..20: mol_type = other RNA
gcagatttcaacagtaactc

SEQ ID NO: 6652 - RNA, 20 nt, synthetic construct
  source 1..20: mol_type = other RNA
atgtgattcataaataatgt

SEQ ID NO: 6653 - RNA, 20 nt, synthetic construct
  source 1..20: mol_type = other RNA
actgcgtgttcgcatcaact

SEQ ID NO: 6654 - RNA, 20 nt, synthetic construct
  source 1..20: mol_type = other RNA
agtgactcatactcaatatt

SEQ ID NO: 6655 - RNA, 20 nt, synthetic construct
  source 1..20: mol_type = other RNA
aggcactagtaatatccttc

SEQ ID NO: 6656 - RNA, 20 nt, synthetic construct
  source 1..20: mol_type = other RNA
taaaactgtagtacgcctga

SEQ ID NO: 6657 - RNA, 20 nt, synthetic construct
  source 1..20: mol_type = other RNA
caaactgtgtatattatgta

SEQ ID NO: 6658 - RNA, 20 nt, synthetic construct
  source 1..20: mol_type = other RNA
aaactgtgtatattatgtat

SEQ ID NO: 6659 - RNA, 20 nt, synthetic construct
  source 1..20: mol_type = other RNA
aactgtgtatattatgtatg

SEQ ID NO: 6660 - RNA, 20 nt, synthetic construct
  source 1..20: mol_type = other RNA
acatcattgttgtacatatg

SEQ ID NO: 6661 - RNA, 20 nt, synthetic construct
  source 1..20: mol_type = other RNA
tgtgtactagattgaacaca

SEQ ID NO: 6662 - RNA, 20 nt, synthetic construct
  source 1..20: mol_type = other RNA
gtacattcctcattagattg

SEQ ID NO: 6663 - RNA, 20 nt, synthetic construct
  source 1..20: mol_type = other RNA
tacattcctcattagattgt

SEQ ID NO: 6664 - RNA, 20 nt, synthetic construct
  source 1..20: mol_type = other RNA
caatctaatgaggaatgtac

SEQ ID NO: 6665 - RNA, 20 nt, synthetic construct
  source 1..20: mol_type = other RNA
ttgaaacccacaatctaatg

SEQ ID NO: 6666 - RNA, 20 nt, synthetic construct
  source 1..20: mol_type = other RNA
ggaaacattcaaattgcaaa

SEQ ID NO: 6667 - RNA, 20 nt, synthetic construct
  source 1..20: mol_type = other RNA
ttggttaagacagagatttc

SEQ ID NO: 6668 - RNA, 20 nt, synthetic construct
  source 1..20: mol_type = other RNA
ttaaccaaacctctctctcc

SEQ ID NO: 6669 - RNA, 20 nt, synthetic construct
  source 1..20: mol_type = other RNA
cgtgcctggagagagaggtt

SEQ ID NO: 6670 - RNA, 20 nt, synthetic construct
  source 1..20: mol_type = other RNA
agaatcgtgcctggagagag

SEQ ID NO: 6671 - RNA, 20 nt, synthetic construct
  source 1..20: mol_type = other RNA
ctcatgtgcagaatcgtgcc

SEQ ID NO: 6672 - RNA, 20 nt, synthetic construct
  source 1..20: mol_type = other RNA
aaaaatgccaaattttgatc

SEQ ID NO: 6673 - RNA, 20 nt, synthetic construct
  source 1..20: mol_type = other RNA
attttgatcaggaatatacc

SEQ ID NO: 6674 - RNA, 20 nt, synthetic construct
  source 1..20: mol_type = other RNA
gtatattcctgatcaaaatt

SEQ ID NO: 6675 - RNA, 20 nt, synthetic construct
  source 1..20: mol_type = other RNA
cctggactactctctttcaa

SEQ ID NO: 6676 - RNA, 20 nt, synthetic construct
  source 1..20: mol_type = other RNA
cctttgaaagagagtagtcc

SEQ ID NO: 6677 - RNA, 20 nt, synthetic construct
  source 1..20: mol_type = other RNA
gcaattgaacatcgtgataa

SEQ ID NO: 6678 - RNA, 20 nt, synthetic construct
  source 1..20: mol_type = other RNA
ataaaggatagcatctattc

SEQ ID NO: 6679 - RNA, 20 nt, synthetic construct
  source 1..20: mol_type = other RNA
gatagcatctattcaggtca

SEQ ID NO: 6680 - RNA, 20 nt, synthetic construct
  source 1..20: mol_type = other RNA
gcatctattcaggtcatgga

SEQ ID NO: 6681 - RNA, 20 nt, synthetic construct
  source 1..20: mol_type = other RNA
attcaggtcatggaaggata

SEQ ID NO: 6682 - RNA, 20 nt, synthetic construct
  source 1..20: mol_type = other RNA
gttgaacttgtgttgaactt

SEQ ID NO: 6683 - RNA, 20 nt, synthetic construct
  source 1..20: mol_type = other RNA
gaacttgtgttgaactttgg

SEQ ID NO: 6684 - RNA, 20 nt, synthetic construct
  source 1..20: mol_type = other RNA
cgtcttcaaataaaaagaca

SEQ ID NO: 6685 - RNA, 20 nt, synthetic construct
  source 1..20: mol_type = other RNA
tgcttaaatttgagagtctc

SEQ ID NO: 6686 - RNA, 20 nt, synthetic construct
  source 1..20: mol_type = other RNA
taaatttgagagtctctgga

SEQ ID NO: 6687 - RNA, 20 nt, synthetic construct
  source 1..20: mol_type = other RNA
atacatcaaactgtgagcag

SEQ ID NO: 6688 - RNA, 20 nt, synthetic construct
  source 1..20: mol_type = other RNA
ctgtgagcagtggttgtctc

SEQ ID NO: 6689 - RNA, 20 nt, synthetic construct
  source 1..20: mol_type = other RNA
cagtggttgtctcaggcaga

SEQ ID NO: 6690 - RNA, 20 nt, synthetic construct
  source 1..20: mol_type = other RNA
agtggttgtctcaggcagaa

SEQ ID NO: 6691 - RNA, 20 nt, synthetic construct
  source 1..20: mol_type = other RNA
ctcaggcagaagggacaacc

SEQ ID NO: 6692 - RNA, 20 nt, synthetic construct
  source 1..20: mol_type = other RNA
tcaggcagaagggacaacca

SEQ ID NO: 6693 - RNA, 20 nt, synthetic construct
  source 1..20: mol_type = other RNA
aagtagaaagtgtaagtccc

SEQ ID NO: 6694 - RNA, 20 nt, synthetic construct
  source 1..20: mol_type = other RNA
ctaattagaaaacacaagaa

SEQ ID NO: 6695 - RNA, 20 nt, synthetic construct
  source 1..20: mol_type = other RNA
aacttgaaacaaaactaaac

SEQ ID NO: 6696 - RNA, 20 nt, synthetic construct
  source 1..20: mol_type = other RNA
gaaacaaaactaaacaggcc

SEQ ID NO: 6697 - RNA, 20 nt, synthetic construct
  source 1..20: mol_type = other RNA
aaaactaaacaggccaggca

SEQ ID NO: 6698 - RNA, 20 nt, synthetic construct
  source 1..20: mol_type = other RNA
actaaacaggccaggcatgg

SEQ ID NO: 6699 - RNA, 20 nt, synthetic construct
  source 1..20: mol_type = other RNA
gcatggtggctcatgcactt

SEQ ID NO: 6700 - RNA, 20 nt, synthetic construct
  source 1..20: mol_type = other RNA
catggtggctcatgcacttt

SEQ ID NO: 6701 - RNA, 20 nt, synthetic construct
  source 1..20: mol_type = other RNA
ggtggctcatgcactttggg

SEQ ID NO: 6702 - RNA, 20 nt, synthetic construct
  source 1..20: mol_type = other RNA
tcatgcactttgggaggccg

SEQ ID NO: 6703 - RNA, 20 nt, synthetic construct
  source 1..20: mol_type = other RNA
ctttgggaggccgaggccaa

SEQ ID NO: 6704 - RNA, 20 nt, synthetic construct
  source 1..20: mol_type = other RNA
ctcaagcgatcctttggcct

SEQ ID NO: 6705 - RNA, 20 nt, synthetic construct
  source 1..20: mol_type = other RNA
ccaaaggatcgcttgagccc

SEQ ID NO: 6706 - RNA, 20 nt, synthetic construct
  source 1..20: mol_type = other RNA
cctgggctcaagcgatcctt

SEQ ID NO: 6707 - RNA, 20 nt, synthetic construct
  source 1..20: mol_type = other RNA
ccaggagtttgagaccagcc

SEQ ID NO: 6708 - RNA, 20 nt, synthetic construct
  source 1..20: mol_type = other RNA
caggagtttgagaccagcct

SEQ ID NO: 6709 - RNA, 20 nt, synthetic construct
  source 1..20: mol_type = other RNA
caggctggtctcaaactcct

SEQ ID NO: 6710 - RNA, 20 nt, synthetic construct
  source 1..20: mol_type = other RNA
ccaggctggtctcaaactcc

SEQ ID NO: 6711 - RNA, 20 nt, synthetic construct
  source 1..20: mol_type = other RNA
tctcactatgttgcccaggc

SEQ ID NO: 6712 - RNA, 20 nt, synthetic construct
  source 1..20: mol_type = other RNA
ggggtctcactatgttgccc

SEQ ID NO: 6713 - RNA, 20 nt, synthetic construct
  source 1..20: mol_type = other RNA
tattttttttgtagagatgg

SEQ ID NO: 6714 - RNA, 20 nt, synthetic construct
  source 1..20: mol_type = other RNA
ttattttttttgtagagatg

SEQ ID NO: 6715 - RNA, 20 nt, synthetic construct
  source 1..20: mol_type = other RNA
tttattttttttgtagagat

SEQ ID NO: 6716 - RNA, 20 nt, synthetic construct
  source 1..20: mol_type = other RNA
ctttattttttttgtagaga

SEQ ID NO: 6717 - RNA, 20 nt, synthetic construct
  source 1..20: mol_type = other RNA
aaaataaagaaaaaattagc

SEQ ID NO: 6718 - RNA, 20 nt, synthetic construct
  source 1..20: mol_type = other RNA
aaataaagaaaaaattagcc

SEQ ID NO: 6719 - RNA, 20 nt, synthetic construct
  source 1..20: mol_type = other RNA
aagaaaaaattagccgggtg

SEQ ID NO: 6720 - RNA, 20 nt, synthetic construct
  source 1..20: mol_type = other RNA
aaaaaattagccgggtgtgg

SEQ ID NO: 6721 - RNA, 20 nt, synthetic construct
  source 1..20: mol_type = other RNA
taggcacgtgccaccacacc

SEQ ID NO: 6722 - RNA, 20 nt, synthetic construct
  source 1..20: mol_type = other RNA
tgcctatcttcccagctgct

SEQ ID NO: 6723 - RNA, 20 nt, synthetic construct
  source 1..20: mol_type = other RNA
gcctatcttcccagctgctt

SEQ ID NO: 6724 - RNA, 20 nt, synthetic construct
  source 1..20: mol_type = other RNA
tatcttcccagctgcttggg

SEQ ID NO: 6725 - RNA, 20 nt, synthetic construct
  source 1..20: mol_type = other RNA
tcccaagcagctgggaagat

SEQ ID NO: 6726 - RNA, 20 nt, synthetic construct
  source 1..20: mol_type = other RNA
cccagctgcttgggaggctg

SEQ ID NO: 6727 - RNA, 20 nt, synthetic construct
  source 1..20: mol_type = other RNA
gctgcttgggaggctgaggc

SEQ ID NO: 6728 - RNA, 20 nt, synthetic construct
  source 1..20: mol_type = other RNA
cctcagcctcccaagcagct

SEQ ID NO: 6729 - RNA, 20 nt, synthetic construct
  source 1..20: mol_type = other RNA
gcctcagcctcccaagcagc

SEQ ID NO: 6730 - RNA, 20 nt, synthetic construct
  source 1..20: mol_type = other RNA
gcttgggaggctgaggcagg

SEQ ID NO: 6731 - RNA, 20 nt, synthetic construct
  source 1..20: mol_type = other RNA
caggaggattgcttgagccc

SEQ ID NO: 6732 - RNA, 20 nt, synthetic construct
  source 1..20: mol_type = other RNA
tgcttgagcccaggagtttg

SEQ ID NO: 6733 - RNA, 20 nt, synthetic construct
  source 1..20: mol_type = other RNA
gcccaggagtttgaggctgc

SEQ ID NO: 6734 - RNA, 20 nt, synthetic construct
  source 1..20: mol_type = other RNA
cccaggagtttgaggctgca

SEQ ID NO: 6735 - RNA, 20 nt, synthetic construct
  source 1..20: mol_type = other RNA
ccctgcagcctcaaactcct

SEQ ID NO: 6736 - RNA, 20 nt, synthetic construct
  source 1..20: mol_type = other RNA
tccctgcagcctcaaactcc

SEQ ID NO: 6737 - RNA, 20 nt, synthetic construct
  source 1..20: mol_type = other RNA
ggaatgcggtggcgcgatca

SEQ ID NO: 6738 - RNA, 20 nt, synthetic construct
  source 1..20: mol_type = other RNA
cgcgccaccgcattccagct

SEQ ID NO: 6739 - RNA, 20 nt, synthetic construct
  source 1..20: mol_type = other RNA
gcgccaccgcattccagctt

SEQ ID NO: 6740 - RNA, 20 nt, synthetic construct
  source 1..20: mol_type = other RNA
tagcccaagctggaatgcgg

SEQ ID NO: 6741 - RNA, 20 nt, synthetic construct
  source 1..20: mol_type = other RNA
ctgtagcccaagctggaatg

SEQ ID NO: 6742 - RNA, 20 nt, synthetic construct
  source 1..20: mol_type = other RNA
tctggctctgtagcccaagc

SEQ ID NO: 6743 - RNA, 20 nt, synthetic construct
  source 1..20: mol_type = other RNA
gttggttttgagaccgggtc

SEQ ID NO: 6744 - RNA, 20 nt, synthetic construct
  source 1..20: mol_type = other RNA
gtttggttggttttgagacc

SEQ ID NO: 6745 - RNA, 20 nt, synthetic construct
  source 1..20: mol_type = other RNA
ggtttggttggttttgagac

SEQ ID NO: 6746 - RNA, 20 nt, synthetic construct
  source 1..20: mol_type = other RNA
gctgttgttgttggtttggt

SEQ ID NO: 6747 - RNA, 20 nt, synthetic construct
  source 1..20: mol_type = other RNA
tactgctgttgttgttggtt

SEQ ID NO: 6748 - RNA, 20 nt, synthetic construct
  source 1..20: mol_type = other RNA
gttgttactgctgttgttgt

SEQ ID NO: 6749 - RNA, 20 nt, synthetic construct
  source 1..20: mol_type = other RNA
taacaacaaaactaagtaaa

SEQ ID NO: 6750 - RNA, 20 nt, synthetic construct
  source 1..20: mol_type = other RNA
tgactttcacaagcaacaat

SEQ ID NO: 6751 - RNA, 20 nt, synthetic construct
  source 1..20: mol_type = other RNA
ctttcacaagcaacaattgg

SEQ ID NO: 6752 - RNA, 20 nt, synthetic construct
  source 1..20: mol_type = other RNA
cacaagcaacaattggagga

SEQ ID NO: 6753 - RNA, 20 nt, synthetic construct
  source 1..20: mol_type = other RNA
gggtttggcatgggtgattt

SEQ ID NO: 6754 - RNA, 20 nt, synthetic construct
  source 1..20: mol_type = other RNA
gtttctgtggggtttggcat

SEQ ID NO: 6755 - RNA, 20 nt, synthetic construct
  source 1..20: mol_type = other RNA
agtttctgtggggtttggca

SEQ ID NO: 6756 - RNA, 20 nt, synthetic construct
  source 1..20: mol_type = other RNA
acagcagtttctgtggggtt

SEQ ID NO: 6757 - RNA, 20 nt, synthetic construct
  source 1..20: mol_type = other RNA
ttggtacagcagtttctgtg

SEQ ID NO: 6758 - RNA, 20 nt, synthetic construct
  source 1..20: mol_type = other RNA
gttggtacagcagtttctgt

SEQ ID NO: 6759 - RNA, 20 nt, synthetic construct
  source 1..20: mol_type = other RNA
cgttggtacagcagtttctg

SEQ ID NO: 6760 - RNA, 20 nt, synthetic construct
  source 1..20: mol_type = other RNA
ggagcacgtgtggagcacgt

SEQ ID NO: 6761 - RNA, 20 nt, synthetic construct
  source 1..20: mol_type = other RNA
tttcatctgtggagcacgtg

SEQ ID NO: 6762 - RNA, 20 nt, synthetic construct
  source 1..20: mol_type = other RNA
tgactgtcttgtttcatctg

SEQ ID NO: 6763 - RNA, 20 nt, synthetic construct
  source 1..20: mol_type = other RNA
gctctgaccactgcccacaa

SEQ ID NO: 6764 - RNA, 20 nt, synthetic construct
  source 1..20: mol_type = other RNA
aaacttaccgttgtgggcag

SEQ ID NO: 6765 - RNA, 20 nt, synthetic construct
  source 1..20: mol_type = other RNA
ttcttgaaacttaccgttgt

SEQ ID NO: 6766 - RNA, 20 nt, synthetic construct
  source 1..20: mol_type = other RNA
cttcttgaaacttaccgttg

SEQ ID NO: 6767 - RNA, 20 nt, synthetic construct
  source 1..20: mol_type = other RNA
taagtttcaagaagttttcc

SEQ ID NO: 6768 - RNA, 20 nt, synthetic construct
  source 1..20: mol_type = other RNA
aagtttcaagaagttttcct

SEQ ID NO: 6769 - RNA, 20 nt, synthetic construct
  source 1..20: mol_type = other RNA
agaagttttcctgggaaatg

SEQ ID NO: 6770 - RNA, 20 nt, synthetic construct
  source 1..20: mol_type = other RNA
gaagttttcctgggaaatgt

SEQ ID NO: 6771 - RNA, 20 nt, synthetic construct
  source 1..20: mol_type = other RNA
tctgatggcccacatttccc

SEQ ID NO: 6772 - RNA, 20 nt, synthetic construct
  source 1..20: mol_type = other RNA
gtgttttatcagcactctga

SEQ ID NO: 6773 - RNA, 20 nt, synthetic construct
  source 1..20: mol_type = other RNA
gagtgctgataaaacactgc

SEQ ID NO: 6774 - RNA, 20 nt, synthetic construct
  source 1..20: mol_type = other RNA
ctgctggcccacctgtcaaa

SEQ ID NO: 6775 - RNA, 20 nt, synthetic construct
  source 1..20: mol_type = other RNA
tgctggcccacctgtcaaat

SEQ ID NO: 6776 - RNA, 20 nt, synthetic construct
  source 1..20: mol_type = other RNA
gctggcccacctgtcaaatg

SEQ ID NO: 6777 - RNA, 20 nt, synthetic construct
  source 1..20: mol_type = other RNA
cctgtcaaatggggcttcac

SEQ ID NO: 6778 - RNA, 20 nt, synthetic construct
  source 1..20: mol_type = other RNA
tgaagccccatttgacaggt

SEQ ID NO: 6779 - RNA, 20 nt, synthetic construct
  source 1..20: mol_type = other RNA
gtgaagccccatttgacagg

SEQ ID NO: 6780 - RNA, 20 nt, synthetic construct
  source 1..20: mol_type = other RNA
cctgtgaagccccatttgac

SEQ ID NO: 6781 - RNA, 20 nt, synthetic construct
  source 1..20: mol_type = other RNA
aacaaagtctgcaactttca

SEQ ID NO: 6782 - RNA, 20 nt, synthetic construct
  source 1..20: mol_type = other RNA
aaagtctgcaactttcaagg

SEQ ID NO: 6783 - RNA, 20 nt, synthetic construct
  source 1..20: mol_type = other RNA
aagtctgcaactttcaaggt

SEQ ID NO: 6784 - RNA, 20 nt, synthetic construct
  source 1..20: mol_type = other RNA
ctgcaactttcaaggtgggc

SEQ ID NO: 6785 - RNA, 20 nt, synthetic construct
  source 1..20: mol_type = other RNA
caggaccagagaagctctcc

SEQ ID NO: 6786 - RNA, 20 nt, synthetic construct
  source 1..20: mol_type = other RNA
gagaagctctccaggtatgc

SEQ ID NO: 6787 - RNA, 20 nt, synthetic construct
  source 1..20: mol_type = other RNA
gcatacctggagagcttctc

SEQ ID NO: 6788 - RNA, 20 nt, synthetic construct
  source 1..20: mol_type = other RNA
ggtatgcaggatagacctcc

SEQ ID NO: 6789 - RNA, 20 nt, synthetic construct
  source 1..20: mol_type = other RNA
gtatgcaggatagacctcca

SEQ ID NO: 6790 - RNA, 20 nt, synthetic construct
  source 1..20: mol_type = other RNA
ggaggtctatcctgcatacc

SEQ ID NO: 6791 - RNA, 20 nt, synthetic construct
  source 1..20: mol_type = other RNA
acataaagggatggccctgg

SEQ ID NO: 6792 - RNA, 20 nt, synthetic construct
  source 1..20: mol_type = other RNA
aacacataaagggatggccc

SEQ ID NO: 6793 - RNA, 20 nt, synthetic construct
  source 1..20: mol_type = other RNA
tattcaaacacataaaggga

SEQ ID NO: 6794 - RNA, 20 nt, synthetic construct
  source 1..20: mol_type = other RNA
gaaatattcaaacacataaa

SEQ ID NO: 6795 - RNA, 20 nt, synthetic construct
  source 1..20: mol_type = other RNA
atgtgtttgaatatttcatc

SEQ ID NO: 6796 - RNA, 20 nt, synthetic construct
  source 1..20: mol_type = other RNA
catcaggattcttcaagagt

SEQ ID NO: 6797 - RNA, 20 nt, synthetic construct
  source 1..20: mol_type = other RNA
gtcatttttttggaggactg

SEQ ID NO: 6798 - RNA, 20 nt, synthetic construct
  source 1..20: mol_type = other RNA
attttgagtcatttttttgg

SEQ ID NO: 6799 - RNA, 20 nt, synthetic construct
  source 1..20: mol_type = other RNA
gaaattttgagtcatttttt

SEQ ID NO: 6800 - RNA, 20 nt, synthetic construct
  source 1..20: mol_type = other RNA
gactcaaaatttcttaagtt

SEQ ID NO: 6801 - RNA, 20 nt, synthetic construct
  source 1..20: mol_type = other RNA
taggttcaagtttctgacat

SEQ ID NO: 6802 - RNA, 20 nt, synthetic construct
  source 1..20: mol_type = other RNA
ttcaagtttctgacatagga

SEQ ID NO: 6803 - RNA, 20 nt, synthetic construct
  source 1..20: mol_type = other RNA
tcaagtttctgacataggat

SEQ ID NO: 6804 - RNA, 20 nt, synthetic construct
  source 1..20: mol_type = other RNA
ctctgccaaaaattagtgaa

SEQ ID NO: 6805 - RNA, 20 nt, synthetic construct
  source 1..20: mol_type = other RNA
tctgccaaaaattagtgaaa

SEQ ID NO: 6806 - RNA, 20 nt, synthetic construct
  source 1..20: mol_type = other RNA
ccaaaaattagtgaaagggc

SEQ ID NO: 6807 - RNA, 20 nt, synthetic construct
  source 1..20: mol_type = other RNA
caaaaattagtgaaagggct

SEQ ID NO: 6808 - RNA, 20 nt, synthetic construct
  source 1..20: mol_type = other RNA
ccagccctttcactaatttt

SEQ ID NO: 6809 - RNA, 20 nt, synthetic construct
  source 1..20: mol_type = other RNA
attagtgaaagggctgggtg

SEQ ID NO: 6810 - RNA, 20 nt, synthetic construct
  source 1..20: mol_type = other RNA
agtgaaagggctgggtgtgg

SEQ ID NO: 6811 - RNA, 20 nt, synthetic construct
  source 1..20: mol_type = other RNA
cgcctgtaatcacaacactt

SEQ ID NO: 6812 - RNA, 20 nt, synthetic construct
  source 1..20: mol_type = other RNA
gcctgtaatcacaacacttt

SEQ ID NO: 6813 - RNA, 20 nt, synthetic construct
  source 1..20: mol_type = other RNA
tgtaatcacaacactttggg

SEQ ID NO: 6814 - RNA, 20 nt, synthetic construct
  source 1..20: mol_type = other RNA
aatcacaacactttgggagg

SEQ ID NO: 6815 - RNA, 20 nt, synthetic construct
  source 1..20: mol_type = other RNA
cacaacactttgggaggtgg

SEQ ID NO: 6816 - RNA, 20 nt, synthetic construct
  source 1..20: mol_type = other RNA
aacactttgggaggtggagg

SEQ ID NO: 6817 - RNA, 20 nt, synthetic construct
  source 1..20: mol_type = other RNA
acactttgggaggtggaggc

SEQ ID NO: 6818 - RNA, 20 nt, synthetic construct
  source 1..20: mol_type = other RNA
ggaggcgggtagatcacctg

SEQ ID NO: 6819 - RNA, 20 nt, synthetic construct
  source 1..20: mol_type = other RNA
cgggtagatcacctgaggtc

SEQ ID NO: 6820 - RNA, 20 nt, synthetic construct
  source 1..20: mol_type = other RNA
cgtctcaaactcctgacctc

SEQ ID NO: 6821 - RNA, 20 nt, synthetic construct
  source 1..20: mol_type = other RNA
tcaggagtttgagacgagcc

SEQ ID NO: 6822 - RNA, 20 nt, synthetic construct
  source 1..20: mol_type = other RNA
tgagacgagcctggccaaca

SEQ ID NO: 6823 - RNA, 20 nt, synthetic construct
  source 1..20: mol_type = other RNA
tgggtttcaccatgttggcc

SEQ ID NO: 6824 - RNA, 20 nt, synthetic construct
  source 1..20: mol_type = other RNA
gagactgggtttcaccatgt

SEQ ID NO: 6825 - RNA, 20 nt, synthetic construct
  source 1..20: mol_type = other RNA
ttgtgtttttagtagagact

SEQ ID NO: 6826 - RNA, 20 nt, synthetic construct
  source 1..20: mol_type = other RNA
tttgtgtttttagtagagac

SEQ ID NO: 6827 - RNA, 20 nt, synthetic construct
  source 1..20: mol_type = other RNA
ctaaaaacacaaaaattagc

SEQ ID NO: 6828 - RNA, 20 nt, synthetic construct
  source 1..20: mol_type = other RNA
taaaaacacaaaaattagct

SEQ ID NO: 6829 - RNA, 20 nt, synthetic construct
  source 1..20: mol_type = other RNA
acacaaaaattagctgggca

SEQ ID NO: 6830 - RNA, 20 nt, synthetic construct
  source 1..20: mol_type = other RNA
cacctgtaatcccagctact

SEQ ID NO: 6831 - RNA, 20 nt, synthetic construct
  source 1..20: mol_type = other RNA
acctgtaatcccagctactt

SEQ ID NO: 6832 - RNA, 20 nt, synthetic construct
  source 1..20: mol_type = other RNA
tgtaatcccagctacttggg

SEQ ID NO: 6833 - RNA, 20 nt, synthetic construct
  source 1..20: mol_type = other RNA
tcccaagtagctgggattac

SEQ ID NO: 6834 - RNA, 20 nt, synthetic construct
  source 1..20: mol_type = other RNA
cccagctacttgggaggctg

SEQ ID NO: 6835 - RNA, 20 nt, synthetic construct
  source 1..20: mol_type = other RNA
agctacttgggaggctgagg

SEQ ID NO: 6836 - RNA, 20 nt, synthetic construct
  source 1..20: mol_type = other RNA
gctacttgggaggctgaggc

SEQ ID NO: 6837 - RNA, 20 nt, synthetic construct
  source 1..20: mol_type = other RNA
cctcagcctcccaagtagct

SEQ ID NO: 6838 - RNA, 20 nt, synthetic construct
  source 1..20: mol_type = other RNA
gcctcagcctcccaagtagc

SEQ ID NO: 6839 - RNA, 20 nt, synthetic construct
  source 1..20: mol_type = other RNA
cgggacaatcacttgaaccc

SEQ ID NO: 6840 - RNA, 20 nt, synthetic construct
  source 1..20: mol_type = other RNA
gacaatcacttgaacccagg

SEQ ID NO: 6841 - RNA, 20 nt, synthetic construct
  source 1..20: mol_type = other RNA
cacttgaacccaggaggcag

SEQ ID NO: 6842 - RNA, 20 nt, synthetic construct
  source 1..20: mol_type = other RNA
cactgcatcctctgcctcct

SEQ ID NO: 6843 - RNA, 20 nt, synthetic construct
  source 1..20: mol_type = other RNA
tcactgcatcctctgcctcc

SEQ ID NO: 6844 - RNA, 20 nt, synthetic construct
  source 1..20: mol_type = other RNA
ggagtgcagtggcacgatct

SEQ ID NO: 6845 - RNA, 20 nt, synthetic construct
  source 1..20: mol_type = other RNA
cgtgccactgcactccagcc

SEQ ID NO: 6846 - RNA, 20 nt, synthetic construct
  source 1..20: mol_type = other RNA
gtgccactgcactccagcct

SEQ ID NO: 6847 - RNA, 20 nt, synthetic construct
  source 1..20: mol_type = other RNA
ttgcccaggctggagtgcag

SEQ ID NO: 6848 - RNA, 20 nt, synthetic construct
  source 1..20: mol_type = other RNA
tttcgctctgttgcccaggc

SEQ ID NO: 6849 - RNA, 20 nt, synthetic construct
  source 1..20: mol_type = other RNA
cgagtttcgctctgttgccc

SEQ ID NO: 6850 - RNA, 20 nt, synthetic construct
  source 1..20: mol_type = other RNA
cgtctcaaaaaaaaagtgaa

SEQ ID NO: 6851 - RNA, 20 nt, synthetic construct
  source 1..20: mol_type = other RNA
gtctcaaaaaaaaagtgaaa

SEQ ID NO: 6852 - RNA, 20 nt, synthetic construct
  source 1..20: mol_type = other RNA
gttgtaagaagcaccccagt

SEQ ID NO: 6853 - RNA, 20 nt, synthetic construct
  source 1..20: mol_type = other RNA
ccagttggagacatgtaaaa

SEQ ID NO: 6854 - RNA, 20 nt, synthetic construct
  source 1..20: mol_type = other RNA
attttacatgtctccaactg

SEQ ID NO: 6855 - RNA, 20 nt, synthetic construct
  source 1..20: mol_type = other RNA
cattttacatgtctccaact

SEQ ID NO: 6856 - RNA, 20 nt, synthetic construct
  source 1..20: mol_type = other RNA
ccattttacatgtctccaac

SEQ ID NO: 6857 - RNA, 20 nt, synthetic construct
  source 1..20: mol_type = other RNA
taatatttccaaatgcttga

SEQ ID NO: 6858 - RNA, 20 nt, synthetic construct
  source 1..20: mol_type = other RNA
ggctttggccttcaagcatt

SEQ ID NO: 6859 - RNA, 20 nt, synthetic construct
  source 1..20: mol_type = other RNA
gtggaatttgcatttggctt

SEQ ID NO: 6860 - RNA, 20 nt, synthetic construct
  source 1..20: mol_type = other RNA
gggcttgtggaatttgcatt

SEQ ID NO: 6861 - RNA, 20 nt, synthetic construct
  source 1..20: mol_type = other RNA
ttgaaaataagaagggcttg

SEQ ID NO: 6862 - RNA, 20 nt, synthetic construct
  source 1..20: mol_type = other RNA
aaattaattgaaaataagaa

SEQ ID NO: 6863 - RNA, 20 nt, synthetic construct
  source 1..20: mol_type = other RNA
gaaattaattgaaaataaga

SEQ ID NO: 6864 - RNA, 20 nt, synthetic construct
  source 1..20: mol_type = other RNA
tgaatcagtgctcagagcta

SEQ ID NO: 6865 - RNA, 20 nt, synthetic construct
  source 1..20: mol_type = other RNA
ttacttcccacctacagatc

SEQ ID NO: 6866 - RNA, 20 nt, synthetic construct
  source 1..20: mol_type = other RNA
tgttagcctgatctgtaggt

SEQ ID NO: 6867 - RNA, 20 nt, synthetic construct
  source 1..20: mol_type = other RNA
ttgttagcctgatctgtagg

SEQ ID NO: 6868 - RNA, 20 nt, synthetic construct
  source 1..20: mol_type = other RNA
tttttgttagcctgatctgt

SEQ ID NO: 6869 - RNA, 20 nt, synthetic construct
  source 1..20: mol_type = other RNA
tcactgatattcttacaggt

SEQ ID NO: 6870 - RNA, 20 nt, synthetic construct
  source 1..20: mol_type = other RNA
acattcactgatattcttac

SEQ ID NO: 6871 - RNA, 20 nt, synthetic construct
  source 1..20: mol_type = other RNA
agaatatcagtgaatgttta

SEQ ID NO: 6872 - RNA, 20 nt, synthetic construct
  source 1..20: mol_type = other RNA
ccgtcatcaccttgaaaaaa

SEQ ID NO: 6873 - RNA, 20 nt, synthetic construct
  source 1..20: mol_type = other RNA
ccattttttcaaggtgatga

SEQ ID NO: 6874 - RNA, 20 nt, synthetic construct
  source 1..20: mol_type = other RNA
tggtgcaatccattttttca

SEQ ID NO: 6875 - RNA, 20 nt, synthetic construct
  source 1..20: mol_type = other RNA
aaggcaggcggtgtaatatg

SEQ ID NO: 6876 - RNA, 20 nt, synthetic construct
  source 1..20: mol_type = other RNA
ctgcctttctcagaccgtcc

SEQ ID NO: 6877 - RNA, 20 nt, synthetic construct
  source 1..20: mol_type = other RNA
gacggtctgagaaaggcagg

SEQ ID NO: 6878 - RNA, 20 nt, synthetic construct
  source 1..20: mol_type = other RNA
caggacggtctgagaaaggc

SEQ ID NO: 6879 - RNA, 20 nt, synthetic construct
  source 1..20: mol_type = other RNA
gcaccaggacggtctgagaa

SEQ ID NO: 6880 - RNA, 20 nt, synthetic construct
  source 1..20: mol_type = other RNA
ttgataaagttgcaccagga

SEQ ID NO: 6881 - RNA, 20 nt, synthetic construct
  source 1..20: mol_type = other RNA
gtgcaactttatcaagtaag

SEQ ID NO: 6882 - RNA, 20 nt, synthetic construct
  source 1..20: mol_type = other RNA
ttacttgataaagttgcacc

SEQ ID NO: 6883 - RNA, 20 nt, synthetic construct
  source 1..20: mol_type = other RNA
ttatcaagtaagaggccaca

SEQ ID NO: 6884 - RNA, 20 nt, synthetic construct
  source 1..20: mol_type = other RNA
aaacaaaaataatgtccttg

SEQ ID NO: 6885 - RNA, 20 nt, synthetic construct
  source 1..20: mol_type = other RNA
ttatttttgtttttaacgtg

SEQ ID NO: 6886 - RNA, 20 nt, synthetic construct
  source 1..20: mol_type = other RNA
caagatagaccctctttttc

SEQ ID NO: 6887 - RNA, 20 nt, synthetic construct
  source 1..20: mol_type = other RNA
aaaataactcctgaaaaaga

SEQ ID NO: 6888 - RNA, 20 nt, synthetic construct
  source 1..20: mol_type = other RNA
gaaaataactcctgaaaaag

SEQ ID NO: 6889 - RNA, 20 nt, synthetic construct
  source 1..20: mol_type = other RNA
gtcatcttgttaaatatatt

SEQ ID NO: 6890 - RNA, 20 nt, synthetic construct
  source 1..20: mol_type = other RNA
ttaacaagatgactaaatct

SEQ ID NO: 6891 - RNA, 20 nt, synthetic construct
  source 1..20: mol_type = other RNA
taacaagatgactaaatcta

SEQ ID NO: 6892 - RNA, 20 nt, synthetic construct
  source 1..20: mol_type = other RNA
caagagaaaaactcagagca

SEQ ID NO: 6893 - RNA, 20 nt, synthetic construct
  source 1..20: mol_type = other RNA
tgtaaacataccagacacac

SEQ ID NO: 6894 - RNA, 20 nt, synthetic construct
  source 1..20: mol_type = other RNA
ataccagacacacaggacac

SEQ ID NO: 6895 - RNA, 20 nt, synthetic construct
  source 1..20: mol_type = other RNA
gacacacaggacacaggaag

SEQ ID NO: 6896 - RNA, 20 nt, synthetic construct
  source 1..20: mol_type = other RNA
cttcctgtgtcctgtgtgtc

SEQ ID NO: 6897 - RNA, 20 nt, synthetic construct
  source 1..20: mol_type = other RNA
caggacacaggaagaggctc

SEQ ID NO: 6898 - RNA, 20 nt, synthetic construct
  source 1..20: mol_type = other RNA
tggttgctgctgccccagaa

SEQ ID NO: 6899 - RNA, 20 nt, synthetic construct
  source 1..20: mol_type = other RNA
aagatcacagttcctttctg

SEQ ID NO: 6900 - RNA, 20 nt, synthetic construct
  source 1..20: mol_type = other RNA
gaagatcacagttcctttct

SEQ ID NO: 6901 - RNA, 20 nt, synthetic construct
  source 1..20: mol_type = other RNA
agaagatcacagttcctttc

SEQ ID NO: 6902 - RNA, 20 nt, synthetic construct
  source 1..20: mol_type = other RNA
tttttcaggctttgattagc

SEQ ID NO: 6903 - RNA, 20 nt, synthetic construct
  source 1..20: mol_type = other RNA
tgatttgggggcgatttttc

SEQ ID NO: 6904 - RNA, 20 nt, synthetic construct
  source 1..20: mol_type = other RNA
cccaaatcaaaacgcatcaa

SEQ ID NO: 6905 - RNA, 20 nt, synthetic construct
  source 1..20: mol_type = other RNA
ccaaatcaaaacgcatcaaa

SEQ ID NO: 6906 - RNA, 20 nt, synthetic construct
  source 1..20: mol_type = other RNA
tttgatgcgttttgatttgg

SEQ ID NO: 6907 - RNA, 20 nt, synthetic construct
  source 1..20: mol_type = other RNA
ctttgatgcgttttgatttg

SEQ ID NO: 6908 - RNA, 20 nt, synthetic construct
  source 1..20: mol_type = other RNA
cctttgatgcgttttgattt

SEQ ID NO: 6909 - RNA, 20 nt, synthetic construct
  source 1..20: mol_type = other RNA
ccctttgatgcgttttgatt

SEQ ID NO: 6910 - RNA, 20 nt, synthetic construct
  source 1..20: mol_type = other RNA
aaaacgcatcaaagggctgc

SEQ ID NO: 6911 - RNA, 20 nt, synthetic construct
  source 1..20: mol_type = other RNA
gcaggtgcacattctgcatg

SEQ ID NO: 6912 - RNA, 20 nt, synthetic construct
  source 1..20: mol_type = other RNA
tgagagaatcagcattatca

SEQ ID NO: 6913 - RNA, 20 nt, synthetic construct
  source 1..20: mol_type = other RNA
atggcaaatagctctcagcc

SEQ ID NO: 6914 - RNA, 20 nt, synthetic construct
  source 1..20: mol_type = other RNA
gctctcagcctggtaagcga

SEQ ID NO: 6915 - RNA, 20 nt, synthetic construct
  source 1..20: mol_type = other RNA
gcctggtaagcgaaggattc

SEQ ID NO: 6916 - RNA, 20 nt, synthetic construct
  source 1..20: mol_type = other RNA
gcctgaatccttcgcttacc

SEQ ID NO: 6917 - RNA, 20 nt, synthetic construct
  source 1..20: mol_type = other RNA
aggattcaggctcctactga

SEQ ID NO: 6918 - RNA, 20 nt, synthetic construct
  source 1..20: mol_type = other RNA
ggattcaggctcctactgaa

SEQ ID NO: 6919 - RNA, 20 nt, synthetic construct
  source 1..20: mol_type = other RNA
tcctactgaagggacaatct

SEQ ID NO: 6920 - RNA, 20 nt, synthetic construct
  source 1..20: mol_type = other RNA
tgaagggacaatctaggtaa

SEQ ID NO: 6921 - RNA, 20 nt, synthetic construct
  source 1..20: mol_type = other RNA
cagattttcttggctaaatg

SEQ ID NO: 6922 - RNA, 20 nt, synthetic construct
  source 1..20: mol_type = other RNA
aaaatctgtaagaaagctat

SEQ ID NO: 6923 - RNA, 20 nt, synthetic construct
  source 1..20: mol_type = other RNA
atctgtaagaaagctattgg

SEQ ID NO: 6924 - RNA, 20 nt, synthetic construct
  source 1..20: mol_type = other RNA
agaaaagacttgaaacagat

SEQ ID NO: 6925 - RNA, 20 nt, synthetic construct
  source 1..20: mol_type = other RNA
attggctgacaaatgccatg

SEQ ID NO: 6926 - RNA, 20 nt, synthetic construct
  source 1..20: mol_type = other RNA
tcggtggctgtagagccaca

SEQ ID NO: 6927 - RNA, 20 nt, synthetic construct
  source 1..20: mol_type = other RNA
ctacagccaccgagtcacag

SEQ ID NO: 6928 - RNA, 20 nt, synthetic construct
  source 1..20: mol_type = other RNA
agccaccgagtcacagtggc

SEQ ID NO: 6929 - RNA, 20 nt, synthetic construct
  source 1..20: mol_type = other RNA
ttcctgccactgtgactcgg

SEQ ID NO: 6930 - RNA, 20 nt, synthetic construct
  source 1..20: mol_type = other RNA
ttcttcctgccactgtgact

SEQ ID NO: 6931 - RNA, 20 nt, synthetic construct
  source 1..20: mol_type = other RNA
gcaggaagaagaaatgcatg

SEQ ID NO: 6932 - RNA, 20 nt, synthetic construct
  source 1..20: mol_type = other RNA
gaagaagaaatgcatgtggc

SEQ ID NO: 6933 - RNA, 20 nt, synthetic construct
  source 1..20: mol_type = other RNA
gaagaaatgcatgtggctgg

SEQ ID NO: 6934 - RNA, 20 nt, synthetic construct
  source 1..20: mol_type = other RNA
aagaaatgcatgtggctggt

SEQ ID NO: 6935 - RNA, 20 nt, synthetic construct
  source 1..20: mol_type = other RNA
gctggtgggcttgttatcac

SEQ ID NO: 6936 - RNA, 20 nt, synthetic construct
  source 1..20: mol_type = other RNA
ctaactgagctccaacacac

SEQ ID NO: 6937 - RNA, 20 nt, synthetic construct
  source 1..20: mol_type = other RNA
ctgtgtgttggagctcagtt

SEQ ID NO: 6938 - RNA, 20 nt, synthetic construct
  source 1..20: mol_type = other RNA
aggtagcagtgcctgtgtgt

SEQ ID NO: 6939 - RNA, 20 nt, synthetic construct
  source 1..20: mol_type = other RNA
ttgaaagttaacagacacta

SEQ ID NO: 6940 - RNA, 20 nt, synthetic construct
  source 1..20: mol_type = other RNA
actgagatttagcaaaaacg

SEQ ID NO: 6941 - RNA, 20 nt, synthetic construct
  source 1..20: mol_type = other RNA
agtgccatttgcatactact

SEQ ID NO: 6942 - RNA, 20 nt, synthetic construct
  source 1..20: mol_type = other RNA
gccatttgcatactacttgg

SEQ ID NO: 6943 - RNA, 20 nt, synthetic construct
  source 1..20: mol_type = other RNA
atttgcatactacttggagg

SEQ ID NO: 6944 - RNA, 20 nt, synthetic construct
  source 1..20: mol_type = other RNA
tttgcatactacttggaggt

SEQ ID NO: 6945 - RNA, 20 nt, synthetic construct
  source 1..20: mol_type = other RNA
ttgcatactacttggaggtg

SEQ ID NO: 6946 - RNA, 20 nt, synthetic construct
  source 1..20: mol_type = other RNA
acctccaagtagtatgcaaa

SEQ ID NO: 6947 - RNA, 20 nt, synthetic construct
  source 1..20: mol_type = other RNA
atactacttggaggtggggc

SEQ ID NO: 6948 - RNA, 20 nt, synthetic construct
  source 1..20: mol_type = other RNA
tactacttggaggtggggct

SEQ ID NO: 6949 - RNA, 20 nt, synthetic construct
  source 1..20: mol_type = other RNA
acttggaggtggggctggga

SEQ ID NO: 6950 - RNA, 20 nt, synthetic construct
  source 1..20: mol_type = other RNA
cttggaggtggggctgggaa

SEQ ID NO: 6951 - RNA, 20 nt, synthetic construct
  source 1..20: mol_type = other RNA
tgagtgtccatctgtttgcc

SEQ ID NO: 6952 - RNA, 20 nt, synthetic construct
  source 1..20: mol_type = other RNA
atgcattccaggcaaacaga

SEQ ID NO: 6953 - RNA, 20 nt, synthetic construct
  source 1..20: mol_type = other RNA
ttatcaactaaatgcattcc

SEQ ID NO: 6954 - RNA, 20 nt, synthetic construct
  source 1..20: mol_type = other RNA
tagttgataatagagtcaga

SEQ ID NO: 6955 - RNA, 20 nt, synthetic construct
  source 1..20: mol_type = other RNA
agttgataatagagtcagat

SEQ ID NO: 6956 - RNA, 20 nt, synthetic construct
  source 1..20: mol_type = other RNA
gttgataatagagtcagatg

SEQ ID NO: 6957 - RNA, 20 nt, synthetic construct
  source 1..20: mol_type = other RNA
ttgataatagagtcagatgg

SEQ ID NO: 6958 - RNA, 20 nt, synthetic construct
  source 1..20: mol_type = other RNA
taatagagtcagatggggga

SEQ ID NO: 6959 - RNA, 20 nt, synthetic construct
  source 1..20: mol_type = other RNA
aatagagtcagatgggggaa

SEQ ID NO: 6960 - RNA, 20 nt, synthetic construct
  source 1..20: mol_type = other RNA
agatgggggaagggaattag

SEQ ID NO: 6961 - RNA, 20 nt, synthetic construct
  source 1..20: mol_type = other RNA
aagggaattagaggaagagc

SEQ ID NO: 6962 - RNA, 20 nt, synthetic construct
  source 1..20: mol_type = other RNA
agggaattagaggaagagca

SEQ ID NO: 6963 - RNA, 20 nt, synthetic construct
  source 1..20: mol_type = other RNA
tagaggaagagcagggtatt

SEQ ID NO: 6964 - RNA, 20 nt, synthetic construct
  source 1..20: mol_type = other RNA
catgcaatctagtaaacttc

SEQ ID NO: 6965 - RNA, 20 nt, synthetic construct
  source 1..20: mol_type = other RNA
acttccggcacaaaaatacc

SEQ ID NO: 6966 - RNA, 20 nt, synthetic construct
  source 1..20: mol_type = other RNA
taagccaggtatttttgtgc

SEQ ID NO: 6967 - RNA, 20 nt, synthetic construct
  source 1..20: mol_type = other RNA
ttgaataatgaaaataagcc

SEQ ID NO: 6968 - RNA, 20 nt, synthetic construct
  source 1..20: mol_type = other RNA
tttgattggtatgtattaat

SEQ ID NO: 6969 - RNA, 20 nt, synthetic construct
  source 1..20: mol_type = other RNA
ttttgattggtatgtattaa

SEQ ID NO: 6970 - RNA, 20 nt, synthetic construct
  source 1..20: mol_type = other RNA
cataccaatcaaaaaataat

SEQ ID NO: 6971 - RNA, 20 nt, synthetic construct
  source 1..20: mol_type = other RNA
ataccaatcaaaaaataatt

SEQ ID NO: 6972 - RNA, 20 nt, synthetic construct
  source 1..20: mol_type = other RNA
taccaatcaaaaaataattg

SEQ ID NO: 6973 - RNA, 20 nt, synthetic construct
  source 1..20: mol_type = other RNA
ttccccaattattttttgat

SEQ ID NO: 6974 - RNA, 20 nt, synthetic construct
  source 1..20: mol_type = other RNA
gtaatcaacagtataagagc

SEQ ID NO: 6975 - RNA, 20 nt, synthetic construct
  source 1..20: mol_type = other RNA
aagagcaggtccatcttcac

SEQ ID NO: 6976 - RNA, 20 nt, synthetic construct
  source 1..20: mol_type = other RNA
agcttgactgccagtgaaga

SEQ ID NO: 6977 - RNA, 20 nt, synthetic construct
  source 1..20: mol_type = other RNA
ttggtgtgctgtattgcacc

SEQ ID NO: 6978 - RNA, 20 nt, synthetic construct
  source 1..20: mol_type = other RNA
atctcatgggttagttaacc

SEQ ID NO: 6979 - RNA, 20 nt, synthetic construct
  source 1..20: mol_type = other RNA
aaattcaaccaaaatctcat

SEQ ID NO: 6980 - RNA, 20 nt, synthetic construct
  source 1..20: mol_type = other RNA
aaaattcaaccaaaatctca

SEQ ID NO: 6981 - RNA, 20 nt, synthetic construct
  source 1..20: mol_type = other RNA
ttgaattttctaagaagtca

SEQ ID NO: 6982 - RNA, 20 nt, synthetic construct
  source 1..20: mol_type = other RNA
aagaagtcacggtttagcac

SEQ ID NO: 6983 - RNA, 20 nt, synthetic construct
  source 1..20: mol_type = other RNA
gtcacggtttagcactggaa

SEQ ID NO: 6984 - RNA, 20 nt, synthetic construct
  source 1..20: mol_type = other RNA
tgtgattgtgtgtgagtgta

SEQ ID NO: 6985 - RNA, 20 nt, synthetic construct
  source 1..20: mol_type = other RNA
gatcagaggtttctgactag

SEQ ID NO: 6986 - RNA, 20 nt, synthetic construct
  source 1..20: mol_type = other RNA
tctgatcactttgtctagcc

SEQ ID NO: 6987 - RNA, 20 nt, synthetic construct
  source 1..20: mol_type = other RNA
ctgatcactttgtctagcct

SEQ ID NO: 6988 - RNA, 20 nt, synthetic construct
  source 1..20: mol_type = other RNA
aggctagacaaagtgatcag

SEQ ID NO: 6989 - RNA, 20 nt, synthetic construct
  source 1..20: mol_type = other RNA
ctttgtctagcctgggatta

SEQ ID NO: 6990 - RNA, 20 nt, synthetic construct
  source 1..20: mol_type = other RNA
tgtctagtttccataatccc

SEQ ID NO: 6991 - RNA, 20 nt, synthetic construct
  source 1..20: mol_type = other RNA
ttatggaaactagacaaaga

SEQ ID NO: 6992 - RNA, 20 nt, synthetic construct
  source 1..20: mol_type = other RNA
tgtatcttacacacatacac

SEQ ID NO: 6993 - RNA, 20 nt, synthetic construct
  source 1..20: mol_type = other RNA
atcttacacacatacacagg

SEQ ID NO: 6994 - RNA, 20 nt, synthetic construct
  source 1..20: mol_type = other RNA
gcatgtgtgtttgtatgtgt

SEQ ID NO: 6995 - RNA, 20 nt, synthetic construct
  source 1..20: mol_type = other RNA
ggcatgtgtgtttgtatgtg

SEQ ID NO: 6996 - RNA, 20 nt, synthetic construct
  source 1..20: mol_type = other RNA
ttgaacaatgatcttttgca

SEQ ID NO: 6997 - RNA, 20 nt, synthetic construct
  source 1..20: mol_type = other RNA
attgaacaatgatcttttgc

SEQ ID NO: 6998 - RNA, 20 nt, synthetic construct
  source 1..20: mol_type = other RNA
aagatcattgttcaatgctg

SEQ ID NO: 6999 - RNA, 20 nt, synthetic construct
  source 1..20: mol_type = other RNA
ccgcagtctgataaatgctg

SEQ ID NO: 7000 - RNA, 20 nt, synthetic construct
  source 1..20: mol_type = other RNA
agtctgataaatgctgtggc

SEQ ID NO: 7001 - RNA, 20 nt, synthetic construct
  source 1..20: mol_type = other RNA
gtctgataaatgctgtggct

SEQ ID NO: 7002 - RNA, 20 nt, synthetic construct
  source 1..20: mol_type = other RNA
caaaaacgttgagccatctg

SEQ ID NO: 7003 - RNA, 20 nt, synthetic construct
  source 1..20: mol_type = other RNA
cacagatggctcaacgtttt

SEQ ID NO: 7004 - RNA, 20 nt, synthetic construct
  source 1..20: mol_type = other RNA
tgggctctggtctccacaga

SEQ ID NO: 7005 - RNA, 20 nt, synthetic construct
  source 1..20: mol_type = other RNA
gtggagaccagagcccactc

SEQ ID NO: 7006 - RNA, 20 nt, synthetic construct
  source 1..20: mol_type = other RNA
ccagagcccactctggcccc

SEQ ID NO: 7007 - RNA, 20 nt, synthetic construct
  source 1..20: mol_type = other RNA
cagagcccactctggcccca

SEQ ID NO: 7008 - RNA, 20 nt, synthetic construct
  source 1..20: mol_type = other RNA
cctggggccagagtgggctc

SEQ ID NO: 7009 - RNA, 20 nt, synthetic construct
  source 1..20: mol_type = other RNA
cccactctggccccagggtg

SEQ ID NO: 7010 - RNA, 20 nt, synthetic construct
  source 1..20: mol_type = other RNA
cctcaccctggggccagagt

SEQ ID NO: 7011 - RNA, 20 nt, synthetic construct
  source 1..20: mol_type = other RNA
acctcaccctggggccagag

SEQ ID NO: 7012 - RNA, 20 nt, synthetic construct
  source 1..20: mol_type = other RNA
cagggtgaggtccctatgac

SEQ ID NO: 7013 - RNA, 20 nt, synthetic construct
  source 1..20: mol_type = other RNA
gtcatagggacctcaccctg

SEQ ID NO: 7014 - RNA, 20 nt, synthetic construct
  source 1..20: mol_type = other RNA
ggtgaggtccctatgacagg

SEQ ID NO: 7015 - RNA, 20 nt, synthetic construct
  source 1..20: mol_type = other RNA
gtgaggtccctatgacaggt

SEQ ID NO: 7016 - RNA, 20 nt, synthetic construct
  source 1..20: mol_type = other RNA
aacagcgcccacctgtcata

SEQ ID NO: 7017 - RNA, 20 nt, synthetic construct
  source 1..20: mol_type = other RNA
gaacagcgcccacctgtcat

SEQ ID NO: 7018 - RNA, 20 nt, synthetic construct
  source 1..20: mol_type = other RNA
cgctgttccgcagccagtgc

SEQ ID NO: 7019 - RNA, 20 nt, synthetic construct
  source 1..20: mol_type = other RNA
gcagccagtgcaggccctgt

SEQ ID NO: 7020 - RNA, 20 nt, synthetic construct
  source 1..20: mol_type = other RNA
cagccagtgcaggccctgtt

SEQ ID NO: 7021 - RNA, 20 nt, synthetic construct
  source 1..20: mol_type = other RNA
aacagggcctgcactggctg

SEQ ID NO: 7022 - RNA, 20 nt, synthetic construct
  source 1..20: mol_type = other RNA
gcaggccctgttgggagtac

SEQ ID NO: 7023 - RNA, 20 nt, synthetic construct
  source 1..20: mol_type = other RNA
cctgttgggagtactggacc

SEQ ID NO: 7024 - RNA, 20 nt, synthetic construct
  source 1..20: mol_type = other RNA
ctggtccagtactcccaaca

SEQ ID NO: 7025 - RNA, 20 nt, synthetic construct
  source 1..20: mol_type = other RNA
cctggtccagtactcccaac

SEQ ID NO: 7026 - RNA, 20 nt, synthetic construct
  source 1..20: mol_type = other RNA
ggtgctccatgctgctgtgc

SEQ ID NO: 7027 - RNA, 20 nt, synthetic construct
  source 1..20: mol_type = other RNA
gtgctccatgctgctgtgca

SEQ ID NO: 7028 - RNA, 20 nt, synthetic construct
  source 1..20: mol_type = other RNA
gcacagcagcatggagcacc

SEQ ID NO: 7029 - RNA, 20 nt, synthetic construct
  source 1..20: mol_type = other RNA
atgctgctgtgcagggtgac

SEQ ID NO: 7030 - RNA, 20 nt, synthetic construct
  source 1..20: mol_type = other RNA
ggtcaccctgcacagcagca

SEQ ID NO: 7031 - RNA, 20 nt, synthetic construct
  source 1..20: mol_type = other RNA
ccggccccatgagcagatcc

SEQ ID NO: 7032 - RNA, 20 nt, synthetic construct
  source 1..20: mol_type = other RNA
cctggatctgctcatggggc

SEQ ID NO: 7033 - RNA, 20 nt, synthetic construct
  source 1..20: mol_type = other RNA
acgacctggatctgctcatg

SEQ ID NO: 7034 - RNA, 20 nt, synthetic construct
  source 1..20: mol_type = other RNA
aacgacctggatctgctcat

SEQ ID NO: 7035 - RNA, 20 nt, synthetic construct
  source 1..20: mol_type = other RNA
caacgacctggatctgctca

SEQ ID NO: 7036 - RNA, 20 nt, synthetic construct
  source 1..20: mol_type = other RNA
ccaggtcgttgaagaattct

SEQ ID NO: 7037 - RNA, 20 nt, synthetic construct
  source 1..20: mol_type = other RNA
caggtcgttgaagaattcta

SEQ ID NO: 7038 - RNA, 20 nt, synthetic construct
  source 1..20: mol_type = other RNA
aggtcgttgaagaattctag

SEQ ID NO: 7039 - RNA, 20 nt, synthetic construct
  source 1..20: mol_type = other RNA
ggtcgttgaagaattctagg

SEQ ID NO: 7040 - RNA, 20 nt, synthetic construct
  source 1..20: mol_type = other RNA
cctagaattcttcaacgacc

SEQ ID NO: 7041 - RNA, 20 nt, synthetic construct
  source 1..20: mol_type = other RNA
ttaagaatgccacacatgct

SEQ ID NO: 7042 - RNA, 20 nt, synthetic construct
  source 1..20: mol_type = other RNA
gatagcacacctagcatgtg

SEQ ID NO: 7043 - RNA, 20 nt, synthetic construct
  source 1..20: mol_type = other RNA
tatcctgagcaactgatgta

SEQ ID NO: 7044 - RNA, 20 nt, synthetic construct
  source 1..20: mol_type = other RNA
tttccttacatcagttgctc

SEQ ID NO: 7045 - RNA, 20 nt, synthetic construct
  source 1..20: mol_type = other RNA
gtaaggaaaaattccattca

SEQ ID NO: 7046 - RNA, 20 nt, synthetic construct
  source 1..20: mol_type = other RNA
atttatatagagaccatgaa

SEQ ID NO: 7047 - RNA, 20 nt, synthetic construct
  source 1..20: mol_type = other RNA
tgtgagtatcccagctactc

SEQ ID NO: 7048 - RNA, 20 nt, synthetic construct
  source 1..20: mol_type = other RNA
gagtatcccagctactcagg

SEQ ID NO: 7049 - RNA, 20 nt, synthetic construct
  source 1..20: mol_type = other RNA
cccagctactcaggaggccg

SEQ ID NO: 7050 - RNA, 20 nt, synthetic construct
  source 1..20: mol_type = other RNA
cctcggcctcctgagtagct

SEQ ID NO: 7051 - RNA, 20 nt, synthetic construct
  source 1..20: mol_type = other RNA
gcctcggcctcctgagtagc

SEQ ID NO: 7052 - RNA, 20 nt, synthetic construct
  source 1..20: mol_type = other RNA
gcagaagaatcgcttgaacc

SEQ ID NO: 7053 - RNA, 20 nt, synthetic construct
  source 1..20: mol_type = other RNA
cagaagaatcgcttgaaccc

SEQ ID NO: 7054 - RNA, 20 nt, synthetic construct
  source 1..20: mol_type = other RNA
aagaatcgcttgaacccggg

SEQ ID NO: 7055 - RNA, 20 nt, synthetic construct
  source 1..20: mol_type = other RNA
aatcgcttgaacccgggagg

SEQ ID NO: 7056 - RNA, 20 nt, synthetic construct
  source 1..20: mol_type = other RNA
acccgggaggcggaagcccc

SEQ ID NO: 7057 - RNA, 20 nt, synthetic construct
  source 1..20: mol_type = other RNA
accaggggcttccgcctccc

SEQ ID NO: 7058 - RNA, 20 nt, synthetic construct
  source 1..20: mol_type = other RNA
aaccaggggcttccgcctcc

SEQ ID NO: 7059 - RNA, 20 nt, synthetic construct
  source 1..20: mol_type = other RNA
cggaagcccctggttccccg

SEQ ID NO: 7060 - RNA, 20 nt, synthetic construct
  source 1..20: mol_type = other RNA
ggaagcccctggttccccgt

SEQ ID NO: 7061 - RNA, 20 nt, synthetic construct
  source 1..20: mol_type = other RNA
gaagcccctggttccccgtg

SEQ ID NO: 7062 - RNA, 20 nt, synthetic construct
  source 1..20: mol_type = other RNA
cacaccccacggggaaccag

SEQ ID NO: 7063 - RNA, 20 nt, synthetic construct
  source 1..20: mol_type = other RNA
gcacaccccacggggaacca

SEQ ID NO: 7064 - RNA, 20 nt, synthetic construct
  source 1..20: mol_type = other RNA
cgcacaccccacggggaacc

SEQ ID NO: 7065 - RNA, 20 nt, synthetic construct
  source 1..20: mol_type = other RNA
cgtggggtgtgcgctcacct

SEQ ID NO: 7066 - RNA, 20 nt, synthetic construct
  source 1..20: mol_type = other RNA
aggtgagcgcacaccccacg

SEQ ID NO: 7067 - RNA, 20 nt, synthetic construct
  source 1..20: mol_type = other RNA
gaggtgagcgcacaccccac

SEQ ID NO: 7068 - RNA, 20 nt, synthetic construct
  source 1..20: mol_type = other RNA
cgaggtgagcgcacacccca

SEQ ID NO: 7069 - RNA, 20 nt, synthetic construct
  source 1..20: mol_type = other RNA
gcgctcacctcggttttcct

SEQ ID NO: 7070 - RNA, 20 nt, synthetic construct
  source 1..20: mol_type = other RNA
cacctcggttttccttggcc

SEQ ID NO: 7071 - RNA, 20 nt, synthetic construct
  source 1..20: mol_type = other RNA
aacctggccaaggaaaaccg

SEQ ID NO: 7072 - RNA, 20 nt, synthetic construct
  source 1..20: mol_type = other RNA
gatggccgacaacctggcca

SEQ ID NO: 7073 - RNA, 20 nt, synthetic construct
  source 1..20: mol_type = other RNA
ctgggagatggccgacaacc

SEQ ID NO: 7074 - RNA, 20 nt, synthetic construct
  source 1..20: mol_type = other RNA
cagctacgactactgggaga

SEQ ID NO: 7075 - RNA, 20 nt, synthetic construct
  source 1..20: mol_type = other RNA
cccagtagtcgtagctgtgc

SEQ ID NO: 7076 - RNA, 20 nt, synthetic construct
  source 1..20: mol_type = other RNA
cctgcacagctacgactact

SEQ ID NO: 7077 - RNA, 20 nt, synthetic construct
  source 1..20: mol_type = other RNA
tcctgcacagctacgactac

SEQ ID NO: 7078 - RNA, 20 nt, synthetic construct
  source 1..20: mol_type = other RNA
gtagctgtgcaggatgctgt

SEQ ID NO: 7079 - RNA, 20 nt, synthetic construct
  source 1..20: mol_type = other RNA
tgctgttggtgatgctgacg

SEQ ID NO: 7080 - RNA, 20 nt, synthetic construct
  source 1..20: mol_type = other RNA
gttggtgatgctgacgtggt

SEQ ID NO: 7081 - RNA, 20 nt, synthetic construct
  source 1..20: mol_type = other RNA
tgacgtggttggccgccatc

SEQ ID NO: 7082 - RNA, 20 nt, synthetic construct
  source 1..20: mol_type = other RNA
cgtggttggccgccatctgg

SEQ ID NO: 7083 - RNA, 20 nt, synthetic construct
  source 1..20: mol_type = other RNA
gccatctggtggatgcgctg

SEQ ID NO: 7084 - RNA, 20 nt, synthetic construct
  source 1..20: mol_type = other RNA
ccatctggtggatgcgctgt

SEQ ID NO: 7085 - RNA, 20 nt, synthetic construct
  source 1..20: mol_type = other RNA
acagcgcatccaccagatgg

SEQ ID NO: 7086 - RNA, 20 nt, synthetic construct
  source 1..20: mol_type = other RNA
cccacagcgcatccaccaga

SEQ ID NO: 7087 - RNA, 20 nt, synthetic construct
  source 1..20: mol_type = other RNA
gcgctgtgggatgctgacga

SEQ ID NO: 7088 - RNA, 20 nt, synthetic construct
  source 1..20: mol_type = other RNA
gggatgctgacgatggtcga

SEQ ID NO: 7089 - RNA, 20 nt, synthetic construct
  source 1..20: mol_type = other RNA
ggatgctgacgatggtcgac

SEQ ID NO: 7090 - RNA, 20 nt, synthetic construct
  source 1..20: mol_type = other RNA
gatgctgacgatggtcgacg

SEQ ID NO: 7091 - RNA, 20 nt, synthetic construct
  source 1..20: mol_type = other RNA
tgacgatggtcgacggggac

SEQ ID NO: 7092 - RNA, 20 nt, synthetic construct
  source 1..20: mol_type = other RNA
gacgatggtcgacggggaca

SEQ ID NO: 7093 - RNA, 20 nt, synthetic construct
  source 1..20: mol_type = other RNA
ggtcgacggggacagggcgc

SEQ ID NO: 7094 - RNA, 20 nt, synthetic construct
  source 1..20: mol_type = other RNA
cggggacagggcgctggcgt

SEQ ID NO: 7095 - RNA, 20 nt, synthetic construct
  source 1..20: mol_type = other RNA
acagggcgctggcgttggag

SEQ ID NO: 7096 - RNA, 20 nt, synthetic construct
  source 1..20: mol_type = other RNA
gaggctgccctgagacccca

SEQ ID NO: 7097 - RNA, 20 nt, synthetic construct
  source 1..20: mol_type = other RNA
gccctgagaccccacggagc

SEQ ID NO: 7098 - RNA, 20 nt, synthetic construct
  source 1..20: mol_type = other RNA
ctgagaccccacggagctgg

SEQ ID NO: 7099 - RNA, 20 nt, synthetic construct
  source 1..20: mol_type = other RNA
tgagaccccacggagctggc

SEQ ID NO: 7100 - RNA, 20 nt, synthetic construct
  source 1..20: mol_type = other RNA
gccagctccgtggggtctca

SEQ ID NO: 7101 - RNA, 20 nt, synthetic construct
  source 1..20: mol_type = other RNA
cgccagctccgtggggtctc

SEQ ID NO: 7102 - RNA, 20 nt, synthetic construct
  source 1..20: mol_type = other RNA
ccccacggagctggcgggag

SEQ ID NO: 7103 - RNA, 20 nt, synthetic construct
  source 1..20: mol_type = other RNA
cccacggagctggcgggaga

SEQ ID NO: 7104 - RNA, 20 nt, synthetic construct
  source 1..20: mol_type = other RNA
ccacggagctggcgggagag

SEQ ID NO: 7105 - RNA, 20 nt, synthetic construct
  source 1..20: mol_type = other RNA
cctctcccgccagctccgtg

SEQ ID NO: 7106 - RNA, 20 nt, synthetic construct
  source 1..20: mol_type = other RNA
ggagctggcgggagaggggt

SEQ ID NO: 7107 - RNA, 20 nt, synthetic construct
  source 1..20: mol_type = other RNA
cccctctcccgccagctccg

SEQ ID NO: 7108 - RNA, 20 nt, synthetic construct
  source 1..20: mol_type = other RNA
gggagaggggttgggagaca

SEQ ID NO: 7109 - RNA, 20 nt, synthetic construct
  source 1..20: mol_type = other RNA
ggagaggggttgggagacat

SEQ ID NO: 7110 - RNA, 20 nt, synthetic construct
  source 1..20: mol_type = other RNA
gagaggggttgggagacatg

SEQ ID NO: 7111 - RNA, 20 nt, synthetic construct
  source 1..20: mol_type = other RNA
agaggggttgggagacatgg

SEQ ID NO: 7112 - RNA, 20 nt, synthetic construct
  source 1..20: mol_type = other RNA
gggttgggagacatggggga

SEQ ID NO: 7113 - RNA, 20 nt, synthetic construct
  source 1..20: mol_type = other RNA
ggttgggagacatgggggat

SEQ ID NO: 7114 - RNA, 20 nt, synthetic construct
  source 1..20: mol_type = other RNA
gttgggagacatgggggatg

SEQ ID NO: 7115 - RNA, 20 nt, synthetic construct
  source 1..20: mol_type = other RNA
ggatggggttccagtgctcc

SEQ ID NO: 7116 - RNA, 20 nt, synthetic construct
  source 1..20: mol_type = other RNA
ggggttccagtgctcctgga

SEQ ID NO: 7117 - RNA, 20 nt, synthetic construct
  source 1..20: mol_type = other RNA
gggttccagtgctcctggaa

SEQ ID NO: 7118 - RNA, 20 nt, synthetic construct
  source 1..20: mol_type = other RNA
ggttccagtgctcctggaag

SEQ ID NO: 7119 - RNA, 20 nt, synthetic construct
  source 1..20: mol_type = other RNA
cagtgctcctggaaggggag

SEQ ID NO: 7120 - RNA, 20 nt, synthetic construct
  source 1..20: mol_type = other RNA
ctctccccttccaggagcac

SEQ ID NO: 7121 - RNA, 20 nt, synthetic construct
  source 1..20: mol_type = other RNA
ttttctacctctccccttcc

SEQ ID NO: 7122 - RNA, 20 nt, synthetic construct
  source 1..20: mol_type = other RNA
gagaggtagaaaaaccagag

SEQ ID NO: 7123 - RNA, 20 nt, synthetic construct
  source 1..20: mol_type = other RNA
gtagaaaaaccagagtggcg

SEQ ID NO: 7124 - RNA, 20 nt, synthetic construct
  source 1..20: mol_type = other RNA
aaaaaccagagtggcgaggt

SEQ ID NO: 7125 - RNA, 20 nt, synthetic construct
  source 1..20: mol_type = other RNA
aaaaccagagtggcgaggtc

SEQ ID NO: 7126 - RNA, 20 nt, synthetic construct
  source 1..20: mol_type = other RNA
tgctcccgacctcgccactc

SEQ ID NO: 7127 - RNA, 20 nt, synthetic construct
  source 1..20: mol_type = other RNA
ggcgaggtcgggagcaagcg

SEQ ID NO: 7128 - RNA, 20 nt, synthetic construct
  source 1..20: mol_type = other RNA
aggtcgggagcaagcgaggc

SEQ ID NO: 7129 - RNA, 20 nt, synthetic construct
  source 1..20: mol_type = other RNA
ggtcgggagcaagcgaggca

SEQ ID NO: 7130 - RNA, 20 nt, synthetic construct
  source 1..20: mol_type = other RNA
agcgaggcagggcagcccct

SEQ ID NO: 7131 - RNA, 20 nt, synthetic construct
  source 1..20: mol_type = other RNA
gcgaggcagggcagcccctt

SEQ ID NO: 7132 - RNA, 20 nt, synthetic construct
  source 1..20: mol_type = other RNA
cgaggcagggcagccccttg

SEQ ID NO: 7133 - RNA, 20 nt, synthetic construct
  source 1..20: mol_type = other RNA
tttgctttctgttccccaag

SEQ ID NO: 7134 - RNA, 20 nt, synthetic construct
  source 1..20: mol_type = other RNA
ctttgctttctgttccccaa

SEQ ID NO: 7135 - RNA, 20 nt, synthetic construct
  source 1..20: mol_type = other RNA
gctttgctttctgttcccca

SEQ ID NO: 7136 - RNA, 20 nt, synthetic construct
  source 1..20: mol_type = other RNA
gaacagaaagcaaagcgcag

SEQ ID NO: 7137 - RNA, 20 nt, synthetic construct
  source 1..20: mol_type = other RNA
gcccagcaccatgcattgtc

SEQ ID NO: 7138 - RNA, 20 nt, synthetic construct
  source 1..20: mol_type = other RNA
gccagacaatgcatggtgct

SEQ ID NO: 7139 - RNA, 20 nt, synthetic construct
  source 1..20: mol_type = other RNA
agccagacaatgcatggtgc

SEQ ID NO: 7140 - RNA, 20 nt, synthetic construct
  source 1..20: mol_type = other RNA
gccgtaagccagacaatgca

SEQ ID NO: 7141 - RNA, 20 nt, synthetic construct
  source 1..20: mol_type = other RNA
ctggcttacggcattgactt

SEQ ID NO: 7142 - RNA, 20 nt, synthetic construct
  source 1..20: mol_type = other RNA
aaagcgaacttactttccac

SEQ ID NO: 7143 - RNA, 20 nt, synthetic construct
  source 1..20: mol_type = other RNA
tactttccactggcccccca

SEQ ID NO: 7144 - RNA, 20 nt, synthetic construct
  source 1..20: mol_type = other RNA
ccactggccccccacggaga

SEQ ID NO: 7145 - RNA, 20 nt, synthetic construct
  source 1..20: mol_type = other RNA
cactggccccccacggagat

SEQ ID NO: 7146 - RNA, 20 nt, synthetic construct
  source 1..20: mol_type = other RNA
actggccccccacggagatg

SEQ ID NO: 7147 - RNA, 20 nt, synthetic construct
  source 1..20: mol_type = other RNA
ccatctccgtggggggccag

SEQ ID NO: 7148 - RNA, 20 nt, synthetic construct
  source 1..20: mol_type = other RNA
ccccccacggagatggggct

SEQ ID NO: 7149 - RNA, 20 nt, synthetic construct
  source 1..20: mol_type = other RNA
cccccacggagatggggctt

SEQ ID NO: 7150 - RNA, 20 nt, synthetic construct
  source 1..20: mol_type = other RNA
ccacggagatggggcttggg

SEQ ID NO: 7151 - RNA, 20 nt, synthetic construct
  source 1..20: mol_type = other RNA
ccaagccccatctccgtggg

SEQ ID NO: 7152 - RNA, 20 nt, synthetic construct
  source 1..20: mol_type = other RNA
cccaagccccatctccgtgg

SEQ ID NO: 7153 - RNA, 20 nt, synthetic construct
  source 1..20: mol_type = other RNA
gcccaagccccatctccgtg

SEQ ID NO: 7154 - RNA, 20 nt, synthetic construct
  source 1..20: mol_type = other RNA
cgcccaagccccatctccgt

SEQ ID NO: 7155 - RNA, 20 nt, synthetic construct
  source 1..20: mol_type = other RNA
ccgcccaagccccatctccg

SEQ ID NO: 7156 - RNA, 20 nt, synthetic construct
  source 1..20: mol_type = other RNA
cagtgagtgccatctgcgtg

SEQ ID NO: 7157 - RNA, 20 nt, synthetic construct
  source 1..20: mol_type = other RNA
ccatctgcgtgaggtgaaac

SEQ ID NO: 7158 - RNA, 20 nt, synthetic construct
  source 1..20: mol_type = other RNA
cctgtttcacctcacgcaga

SEQ ID NO: 7159 - RNA, 20 nt, synthetic construct
  source 1..20: mol_type = other RNA
ggtgacatgaacgtgttttc

SEQ ID NO: 7160 - RNA, 20 nt, synthetic construct
  source 1..20: mol_type = other RNA
gtgactgcagagagaagcaa

SEQ ID NO: 7161 - RNA, 20 nt, synthetic construct
  source 1..20: mol_type = other RNA
gaagcaaaggcagacactgc

SEQ ID NO: 7162 - RNA, 20 nt, synthetic construct
  source 1..20: mol_type = other RNA
aggcagacactgcaggaaaa

SEQ ID NO: 7163 - RNA, 20 nt, synthetic construct
  source 1..20: mol_type = other RNA
caggtcacctctggtcccca

SEQ ID NO: 7164 - RNA, 20 nt, synthetic construct
  source 1..20: mol_type = other RNA
gggttaatgcaggtcacctc

SEQ ID NO: 7165 - RNA, 20 nt, synthetic construct
  source 1..20: mol_type = other RNA
ctgcattaaccccaaagcaa

SEQ ID NO: 7166 - RNA, 20 nt, synthetic construct
  source 1..20: mol_type = other RNA
cattgctttggggttaatgc

SEQ ID NO: 7167 - RNA, 20 nt, synthetic construct
  source 1..20: mol_type = other RNA
ccaaagcaatggagtctacc

SEQ ID NO: 7168 - RNA, 20 nt, synthetic construct
  source 1..20: mol_type = other RNA
tggtagactccattgctttg

SEQ ID NO: 7169 - RNA, 20 nt, synthetic construct
  source 1..20: mol_type = other RNA
ctggtagactccattgcttt

SEQ ID NO: 7170 - RNA, 20 nt, synthetic construct
  source 1..20: mol_type = other RNA
cctggtagactccattgctt

SEQ ID NO: 7171 - RNA, 20 nt, synthetic construct
  source 1..20: mol_type = other RNA
aggtgcttcacaaatttgac

SEQ ID NO: 7172 - RNA, 20 nt, synthetic construct
  source 1..20: mol_type = other RNA
ggtgcttcacaaatttgaca

SEQ ID NO: 7173 - RNA, 20 nt, synthetic construct
  source 1..20: mol_type = other RNA
tgtcaaatttgtgaagcacc

SEQ ID NO: 7174 - RNA, 20 nt, synthetic construct
  source 1..20: mol_type = other RNA
cagggagacaagtgaaatta

SEQ ID NO: 7175 - RNA, 20 nt, synthetic construct
  source 1..20: mol_type = other RNA
agcactaatcgactatttca

SEQ ID NO: 7176 - RNA, 20 nt, synthetic construct
  source 1..20: mol_type = other RNA
cttttgaatactttacagcg

SEQ ID NO: 7177 - RNA, 20 nt, synthetic construct
  source 1..20: mol_type = other RNA
gcggatgtttcgactcaaaa

SEQ ID NO: 7178 - RNA, 20 nt, synthetic construct
  source 1..20: mol_type = other RNA
ggcggatgtttcgactcaaa

SEQ ID NO: 7179 - RNA, 20 nt, synthetic construct
  source 1..20: mol_type = other RNA
gtcgaaacatccgccagtac

SEQ ID NO: 7180 - RNA, 20 nt, synthetic construct
  source 1..20: mol_type = other RNA
gaaacatccgccagtacagg

SEQ ID NO: 7181 - RNA, 20 nt, synthetic construct
  source 1..20: mol_type = other RNA
aaacatccgccagtacagga

SEQ ID NO: 7182 - RNA, 20 nt, synthetic construct
  source 1..20: mol_type = other RNA
tccgccagtacaggagggcc

SEQ ID NO: 7183 - RNA, 20 nt, synthetic construct
  source 1..20: mol_type = other RNA
gcctggccctcctgtactgg

SEQ ID NO: 7184 - RNA, 20 nt, synthetic construct
  source 1..20: mol_type = other RNA
gatgcctggccctcctgtac

SEQ ID NO: 7185 - RNA, 20 nt, synthetic construct
  source 1..20: mol_type = other RNA
ggccaggcatcggtaactgc

SEQ ID NO: 7186 - RNA, 20 nt, synthetic construct
  source 1..20: mol_type = other RNA
cgcctgcagttaccgatgcc

SEQ ID NO: 7187 - RNA, 20 nt, synthetic construct
  source 1..20: mol_type = other RNA
ctgcaggcgaaaagagaaac

SEQ ID NO: 7188 - RNA, 20 nt, synthetic construct
  source 1..20: mol_type = other RNA
aagagaaacaggcccagaag

SEQ ID NO: 7189 - RNA, 20 nt, synthetic construct
  source 1..20: mol_type = other RNA
cgacgcactcagccgcttct

SEQ ID NO: 7190 - RNA, 20 nt, synthetic construct
  source 1..20: mol_type = other RNA
acgacgcactcagccgcttc

SEQ ID NO: 7191 - RNA, 20 nt, synthetic construct
  source 1..20: mol_type = other RNA
acatttttgttgttgttcta

SEQ ID NO: 7192 - RNA, 20 nt, synthetic construct
  source 1..20: mol_type = other RNA
acaataccttgtttctacat

SEQ ID NO: 7193 - RNA, 20 nt, synthetic construct
  source 1..20: mol_type = other RNA
ctttgtatgttagaagacat

SEQ ID NO: 7194 - RNA, 20 nt, synthetic construct
  source 1..20: mol_type = other RNA
tttgtatgttagaagacatt

SEQ ID NO: 7195 - RNA, 20 nt, synthetic construct
  source 1..20: mol_type = other RNA
acactatgcctttcagcacc

SEQ ID NO: 7196 - RNA, 20 nt, synthetic construct
  source 1..20: mol_type = other RNA
ttggcaaaccaggtgctgaa

SEQ ID NO: 7197 - RNA, 20 nt, synthetic construct
  source 1..20: mol_type = other RNA
agcacctggtttgccaatga

SEQ ID NO: 7198 - RNA, 20 nt, synthetic construct
  source 1..20: mol_type = other RNA
tttgccaatgatggcatgcg

SEQ ID NO: 7199 - RNA, 20 nt, synthetic construct
  source 1..20: mol_type = other RNA
ccaatgatggcatgcgaggc

SEQ ID NO: 7200 - RNA, 20 nt, synthetic construct
  source 1..20: mol_type = other RNA
caatgatggcatgcgaggct

SEQ ID NO: 7201 - RNA, 20 nt, synthetic construct
  source 1..20: mol_type = other RNA
aatgatggcatgcgaggctg

SEQ ID NO: 7202 - RNA, 20 nt, synthetic construct
  source 1..20: mol_type = other RNA
ccagcctcgcatgccatcat

SEQ ID NO: 7203 - RNA, 20 nt, synthetic construct
  source 1..20: mol_type = other RNA
gctggggctgctattctaag

SEQ ID NO: 7204 - RNA, 20 nt, synthetic construct
  source 1..20: mol_type = other RNA
gctgctattctaagcggaga

SEQ ID NO: 7205 - RNA, 20 nt, synthetic construct
  source 1..20: mol_type = other RNA
ctgctattctaagcggagat

SEQ ID NO: 7206 - RNA, 20 nt, synthetic construct
  source 1..20: mol_type = other RNA
acaaacaactggctgcatta

SEQ ID NO: 7207 - RNA, 20 nt, synthetic construct
  source 1..20: mol_type = other RNA
gcagccagttgtttgtcttc

SEQ ID NO: 7208 - RNA, 20 nt, synthetic construct
  source 1..20: mol_type = other RNA
cagttgtttgtcttctggtg

SEQ ID NO: 7209 - RNA, 20 nt, synthetic construct
  source 1..20: mol_type = other RNA
cacaccagaagacaaacaac

SEQ ID NO: 7210 - RNA, 20 nt, synthetic construct
  source 1..20: mol_type = other RNA
tttgtcttctggtgtggcat

SEQ ID NO: 7211 - RNA, 20 nt, synthetic construct
  source 1..20: mol_type = other RNA
ttgtcttctggtgtggcatt

SEQ ID NO: 7212 - RNA, 20 nt, synthetic construct
  source 1..20: mol_type = other RNA
tgtcttctggtgtggcattg

SEQ ID NO: 7213 - RNA, 20 nt, synthetic construct
  source 1..20: mol_type = other RNA
gtgtggcattggggcctgag

SEQ ID NO: 7214 - RNA, 20 nt, synthetic construct
  source 1..20: mol_type = other RNA
tgtggcattggggcctgagt

SEQ ID NO: 7215 - RNA, 20 nt, synthetic construct
  source 1..20: mol_type = other RNA
atgagactaaaaacccactc

SEQ ID NO: 7216 - RNA, 20 nt, synthetic construct
  source 1..20: mol_type = other RNA
atagcataccttagaaaaag

SEQ ID NO: 7217 - RNA, 20 nt, synthetic construct
  source 1..20: mol_type = other RNA
tagcataccttagaaaaagc

SEQ ID NO: 7218 - RNA, 20 nt, synthetic construct
  source 1..20: mol_type = other RNA
agcataccttagaaaaagcg

SEQ ID NO: 7219 - RNA, 20 nt, synthetic construct
  source 1..20: mol_type = other RNA
ataccttagaaaaagcgggg

SEQ ID NO: 7220 - RNA, 20 nt, synthetic construct
  source 1..20: mol_type = other RNA
ccttagaaaaagcggggagg

SEQ ID NO: 7221 - RNA, 20 nt, synthetic construct
  source 1..20: mol_type = other RNA
cctcctccccgctttttcta

SEQ ID NO: 7222 - RNA, 20 nt, synthetic construct
  source 1..20: mol_type = other RNA
tattaacagaacttctatga

SEQ ID NO: 7223 - RNA, 20 nt, synthetic construct
  source 1..20: mol_type = other RNA
gggggatgaacactggttcc

SEQ ID NO: 7224 - RNA, 20 nt, synthetic construct
  source 1..20: mol_type = other RNA
ggatgaacactggttcctgg

SEQ ID NO: 7225 - RNA, 20 nt, synthetic construct
  source 1..20: mol_type = other RNA
gatgaacactggttcctggt

SEQ ID NO: 7226 - RNA, 20 nt, synthetic construct
  source 1..20: mol_type = other RNA
atgaacactggttcctggtg

SEQ ID NO: 7227 - RNA, 20 nt, synthetic construct
  source 1..20: mol_type = other RNA
tgaacactggttcctggtgg

SEQ ID NO: 7228 - RNA, 20 nt, synthetic construct
  source 1..20: mol_type = other RNA
cactggttcctggtggggga

SEQ ID NO: 7229 - RNA, 20 nt, synthetic construct
  source 1..20: mol_type = other RNA
ttcctggtgggggatggtgc

SEQ ID NO: 7230 - RNA, 20 nt, synthetic construct
  source 1..20: mol_type = other RNA
agcctgcaccatcccccacc

SEQ ID NO: 7231 - RNA, 20 nt, synthetic construct
  source 1..20: mol_type = other RNA
aggaatgtgtggaagcacta

SEQ ID NO: 7232 - RNA, 20 nt, synthetic construct
  source 1..20: mol_type = other RNA
ggggaggagtgaggaatgtg

SEQ ID NO: 7233 - RNA, 20 nt, synthetic construct
  source 1..20: mol_type = other RNA
gctggatgaggggaggagtg

SEQ ID NO: 7234 - RNA, 20 nt, synthetic construct
  source 1..20: mol_type = other RNA
cctcatccagcaagaaaaca

SEQ ID NO: 7235 - RNA, 20 nt, synthetic construct
  source 1..20: mol_type = other RNA
gtgttttcttgctggatgag

SEQ ID NO: 7236 - RNA, 20 nt, synthetic construct
  source 1..20: mol_type = other RNA
cgtgttttcttgctggatga

SEQ ID NO: 7237 - RNA, 20 nt, synthetic construct
  source 1..20: mol_type = other RNA
ccgtgttttcttgctggatg

SEQ ID NO: 7238 - RNA, 20 nt, synthetic construct
  source 1..20: mol_type = other RNA
taagcaccgtgttttcttgc

SEQ ID NO: 7239 - RNA, 20 nt, synthetic construct
  source 1..20: mol_type = other RNA
cagaaacagtagagctcatc

SEQ ID NO: 7240 - RNA, 20 nt, synthetic construct
  source 1..20: mol_type = other RNA
gtttctgaatacatcgtata

SEQ ID NO: 7241 - RNA, 20 nt, synthetic construct
  source 1..20: mol_type = other RNA
atacatcgtataaggagatt

SEQ ID NO: 7242 - RNA, 20 nt, synthetic construct
  source 1..20: mol_type = other RNA
ataaggagatttggattcca

SEQ ID NO: 7243 - RNA, 20 nt, synthetic construct
  source 1..20: mol_type = other RNA
taaggagatttggattccat

SEQ ID NO: 7244 - RNA, 20 nt, synthetic construct
  source 1..20: mol_type = other RNA
aaggagatttggattccatg

SEQ ID NO: 7245 - RNA, 20 nt, synthetic construct
  source 1..20: mol_type = other RNA
tgcaatggaacaaggcccca

SEQ ID NO: 7246 - RNA, 20 nt, synthetic construct
  source 1..20: mol_type = other RNA
tgtggaaatgcaatggaaca

SEQ ID NO: 7247 - RNA, 20 nt, synthetic construct
  source 1..20: mol_type = other RNA
tatcgagtgtggaaatgcaa

SEQ ID NO: 7248 - RNA, 20 nt, synthetic construct
  source 1..20: mol_type = other RNA
gcattgtcgtttatcgagtg

SEQ ID NO: 7249 - RNA, 20 nt, synthetic construct
  source 1..20: mol_type = other RNA
tcaggtggaaaagtttggaa

SEQ ID NO: 7250 - RNA, 20 nt, synthetic construct
  source 1..20: mol_type = other RNA
gttgatcaggtggaaaagtt

SEQ ID NO: 7251 - RNA, 20 nt, synthetic construct
  source 1..20: mol_type = other RNA
tattaactctgttgatcagg

SEQ ID NO: 7252 - RNA, 20 nt, synthetic construct
  source 1..20: mol_type = other RNA
ctgtattaactctgttgatc

SEQ ID NO: 7253 - RNA, 20 nt, synthetic construct
  source 1..20: mol_type = other RNA
aaacaatagttttttttaaa

SEQ ID NO: 7254 - RNA, 20 nt, synthetic construct
  source 1..20: mol_type = other RNA
tttaaaaaaaactattgttt

SEQ ID NO: 7255 - RNA, 20 nt, synthetic construct
  source 1..20: mol_type = other RNA
agagttgggtttctcaaata

SEQ ID NO: 7256 - RNA, 20 nt, synthetic construct
  source 1..20: mol_type = other RNA
ggattttagaagtcagagtt

SEQ ID NO: 7257 - RNA, 20 nt, synthetic construct
  source 1..20: mol_type = other RNA
aggattttagaagtcagagt

SEQ ID NO: 7258 - RNA, 20 nt, synthetic construct
  source 1..20: mol_type = other RNA
ggatggccgggtctgttcaa

SEQ ID NO: 7259 - RNA, 20 nt, synthetic construct
  source 1..20: mol_type = other RNA
aatctattacaaggatggcc

SEQ ID NO: 7260 - RNA, 20 nt, synthetic construct
  source 1..20: mol_type = other RNA
aaatctattacaaggatggc

SEQ ID NO: 7261 - RNA, 20 nt, synthetic construct
  source 1..20: mol_type = other RNA
tataaaatctattacaagga

SEQ ID NO: 7262 - RNA, 20 nt, synthetic construct
  source 1..20: mol_type = other RNA
taattataaaatctattaca

SEQ ID NO: 7263 - RNA, 20 nt, synthetic construct
  source 1..20: mol_type = other RNA
tcactgggacaatatagctg

SEQ ID NO: 7264 - RNA, 20 nt, synthetic construct
  source 1..20: mol_type = other RNA
atcactgggacaatatagct

SEQ ID NO: 7265 - RNA, 20 nt, synthetic construct
  source 1..20: mol_type = other RNA
catcactgggacaatatagc

SEQ ID NO: 7266 - RNA, 20 nt, synthetic construct
  source 1..20: mol_type = other RNA
tgtactgcagcttcatcact

SEQ ID NO: 7267 - RNA, 20 nt, synthetic construct
  source 1..20: mol_type = other RNA
gtgtactgcagcttcatcac

SEQ ID NO: 7268 - RNA, 20 nt, synthetic construct
  source 1..20: mol_type = other RNA
gctgcagtacacacataatt

SEQ ID NO: 7269 - RNA, 20 nt, synthetic construct
  source 1..20: mol_type = other RNA
ataatttggaagaacgtatc

SEQ ID NO: 7270 - RNA, 20 nt, synthetic construct
  source 1..20: mol_type = other RNA
agaacgtatctggaaagaaa

SEQ ID NO: 7271 - RNA, 20 nt, synthetic construct
  source 1..20: mol_type = other RNA
gaacgtatctggaaagaaaa

SEQ ID NO: 7272 - RNA, 20 nt, synthetic construct
  source 1..20: mol_type = other RNA
gaagcataaagcagatgcaa

SEQ ID NO: 7273 - RNA, 20 nt, synthetic construct
  source 1..20: mol_type = other RNA
agcttcttgcataaaataat

SEQ ID NO: 7274 - RNA, 20 nt, synthetic construct
  source 1..20: mol_type = other RNA
ataaaataatcggcactgcg

SEQ ID NO: 7275 - RNA, 20 nt, synthetic construct
  source 1..20: mol_type = other RNA
tcggcactgcgaggcctaca

SEQ ID NO: 7276 - RNA, 20 nt, synthetic construct
  source 1..20: mol_type = other RNA
taatatcattctctccttgt

SEQ ID NO: 7277 - RNA, 20 nt, synthetic construct
  source 1..20: mol_type = other RNA
aatgatattaaacgtcatta

SEQ ID NO: 7278 - RNA, 20 nt, synthetic construct
  source 1..20: mol_type = other RNA
cttcctttcactcaaactta

SEQ ID NO: 7279 - RNA, 20 nt, synthetic construct
  source 1..20: mol_type = other RNA
cttaagtttgagtgaaagga

SEQ ID NO: 7280 - RNA, 20 nt, synthetic construct
  source 1..20: mol_type = other RNA
gtgccttaagtttgagtgaa

SEQ ID NO: 7281 - RNA, 20 nt, synthetic construct
  source 1..20: mol_type = other RNA
tttaaaaactctgcttaatg

SEQ ID NO: 7282 - RNA, 20 nt, synthetic construct
  source 1..20: mol_type = other RNA
gtgcggcctttttttcccct

SEQ ID NO: 7283 - RNA, 20 nt, synthetic construct
  source 1..20: mol_type = other RNA
agtgcggcctttttttcccc

SEQ ID NO: 7284 - RNA, 20 nt, synthetic construct
  source 1..20: mol_type = other RNA
aaaggccgcactgtagctga

SEQ ID NO: 7285 - RNA, 20 nt, synthetic construct
  source 1..20: mol_type = other RNA
ggccgcactgtagctgaagg

SEQ ID NO: 7286 - RNA, 20 nt, synthetic construct
  source 1..20: mol_type = other RNA
ggccaccttcagctacagtg

SEQ ID NO: 7287 - RNA, 20 nt, synthetic construct
  source 1..20: mol_type = other RNA
agctgaaggtggccacacca

SEQ ID NO: 7288 - RNA, 20 nt, synthetic construct
  source 1..20: mol_type = other RNA
ggggcatgggcaccttggtg

SEQ ID NO: 7289 - RNA, 20 nt, synthetic construct
  source 1..20: mol_type = other RNA
tggaaggggcatgggcacct

SEQ ID NO: 7290 - RNA, 20 nt, synthetic construct
  source 1..20: mol_type = other RNA
tgctcaggtggaaggggcat

SEQ ID NO: 7291 - RNA, 20 nt, synthetic construct
  source 1..20: mol_type = other RNA
ctgctcaggtggaaggggca

SEQ ID NO: 7292 - RNA, 20 nt, synthetic construct
  source 1..20: mol_type = other RNA
agaagctgctcaggtggaag

SEQ ID NO: 7293 - RNA, 20 nt, synthetic construct
  source 1..20: mol_type = other RNA
cagaagctgctcaggtggaa

SEQ ID NO: 7294 - RNA, 20 nt, synthetic construct
  source 1..20: mol_type = other RNA
acagaagctgctcaggtgga

SEQ ID NO: 7295 - RNA, 20 nt, synthetic construct
  source 1..20: mol_type = other RNA
cagaacagaagctgctcagg

SEQ ID NO: 7296 - RNA, 20 nt, synthetic construct
  source 1..20: mol_type = other RNA
agacagaacagaagctgctc

SEQ ID NO: 7297 - RNA, 20 nt, synthetic construct
  source 1..20: mol_type = other RNA
acgcttttaaatgtggtgag

SEQ ID NO: 7298 - RNA, 20 nt, synthetic construct
  source 1..20: mol_type = other RNA
gacgcttttaaatgtggtga

SEQ ID NO: 7299 - RNA, 20 nt, synthetic construct
  source 1..20: mol_type = other RNA
agacgcttttaaatgtggtg

SEQ ID NO: 7300 - RNA, 20 nt, synthetic construct
  source 1..20: mol_type = other RNA
agttcagacgcttttaaatg

SEQ ID NO: 7301 - RNA, 20 nt, synthetic construct
  source 1..20: mol_type = other RNA
tctgcctcttgcagtccctg

SEQ ID NO: 7302 - RNA, 20 nt, synthetic construct
  source 1..20: mol_type = other RNA
cttgcagtccctgtggccgt

SEQ ID NO: 7303 - RNA, 20 nt, synthetic construct
  source 1..20: mol_type = other RNA
acggccacagggactgcaag

SEQ ID NO: 7304 - RNA, 20 nt, synthetic construct
  source 1..20: mol_type = other RNA
tccctgtggccgttggagcc

SEQ ID NO: 7305 - RNA, 20 nt, synthetic construct
  source 1..20: mol_type = other RNA
tccaggctccaacggccaca

SEQ ID NO: 7306 - RNA, 20 nt, synthetic construct
  source 1..20: mol_type = other RNA
ctccaggctccaacggccac

SEQ ID NO: 7307 - RNA, 20 nt, synthetic construct
  source 1..20: mol_type = other RNA
ccgttggagcctggagacca

SEQ ID NO: 7308 - RNA, 20 nt, synthetic construct
  source 1..20: mol_type = other RNA
ccgtggtctccaggctccaa

SEQ ID NO: 7309 - RNA, 20 nt, synthetic construct
  source 1..20: mol_type = other RNA
ggagaccacggcttcgtctg

SEQ ID NO: 7310 - RNA, 20 nt, synthetic construct
  source 1..20: mol_type = other RNA
cagacgaagccgtggtctcc

SEQ ID NO: 7311 - RNA, 20 nt, synthetic construct
  source 1..20: mol_type = other RNA
cacggccgcagacgaagccg

SEQ ID NO: 7312 - RNA, 20 nt, synthetic construct
  source 1..20: mol_type = other RNA
tcgtctgcggccgtgacttg

SEQ ID NO: 7313 - RNA, 20 nt, synthetic construct
  source 1..20: mol_type = other RNA
tctgcggccgtgacttgtgg

SEQ ID NO: 7314 - RNA, 20 nt, synthetic construct
  source 1..20: mol_type = other RNA
ctgcggccgtgacttgtgga

SEQ ID NO: 7315 - RNA, 20 nt, synthetic construct
  source 1..20: mol_type = other RNA
tgcggccgtgacttgtggag

SEQ ID NO: 7316 - RNA, 20 nt, synthetic construct
  source 1..20: mol_type = other RNA
acattcccctccacaagtca

SEQ ID NO: 7317 - RNA, 20 nt, synthetic construct
  source 1..20: mol_type = other RNA
aacacacatctttgagaaat

SEQ ID NO: 7318 - RNA, 20 nt, synthetic construct
  source 1..20: mol_type = other RNA
tctttgagaaattggccacc

SEQ ID NO: 7319 - RNA, 20 nt, synthetic construct
  source 1..20: mol_type = other RNA
gggctgctcgcttcaccagg

SEQ ID NO: 7320 - RNA, 20 nt, synthetic construct
  source 1..20: mol_type = other RNA
gatgggctgctcgcttcacc

SEQ ID NO: 7321 - RNA, 20 nt, synthetic construct
  source 1..20: mol_type = other RNA
tacgtatgtatgtatgtgat

SEQ ID NO: 7322 - RNA, 20 nt, synthetic construct
  source 1..20: mol_type = other RNA
ctacgtatgtatgtatgtga

SEQ ID NO: 7323 - RNA, 20 nt, synthetic construct
  source 1..20: mol_type = other RNA
atacatacgtagaatatctt

SEQ ID NO: 7324 - RNA, 20 nt, synthetic construct
  source 1..20: mol_type = other RNA
acagtctgaacacatgcttg

SEQ ID NO: 7325 - RNA, 20 nt, synthetic construct
  source 1..20: mol_type = other RNA
gcatgtgttcagactgtgct

SEQ ID NO: 7326 - RNA, 20 nt, synthetic construct
  source 1..20: mol_type = other RNA
gctaggttagagacagagct

SEQ ID NO: 7327 - RNA, 20 nt, synthetic construct
  source 1..20: mol_type = other RNA
ctaggttagagacagagctt

SEQ ID NO: 7328 - RNA, 20 nt, synthetic construct
  source 1..20: mol_type = other RNA
taggttagagacagagcttg

SEQ ID NO: 7329 - RNA, 20 nt, synthetic construct
  source 1..20: mol_type = other RNA
aggttagagacagagcttgg

SEQ ID NO: 7330 - RNA, 20 nt, synthetic construct
  source 1..20: mol_type = other RNA
gggggtgctcaatttcattt

SEQ ID NO: 7331 - RNA, 20 nt, synthetic construct
  source 1..20: mol_type = other RNA
aatttcattttggttttaat

SEQ ID NO: 7332 - RNA, 20 nt, synthetic construct
  source 1..20: mol_type = other RNA
atttcattttggttttaatt

SEQ ID NO: 7333 - RNA, 20 nt, synthetic construct
  source 1..20: mol_type = other RNA
attttggttttaattgggaa

SEQ ID NO: 7334 - RNA, 20 nt, synthetic construct
  source 1..20: mol_type = other RNA
aagagcatcaacaaaccgtg

SEQ ID NO: 7335 - RNA, 20 nt, synthetic construct
  source 1..20: mol_type = other RNA
accgtgaggtctccgccgtg

SEQ ID NO: 7336 - RNA, 20 nt, synthetic construct
  source 1..20: mol_type = other RNA
gcctcacggcggagacctca

SEQ ID NO: 7337 - RNA, 20 nt, synthetic construct
  source 1..20: mol_type = other RNA
ctccgccgtgaggctgcagc

SEQ ID NO: 7338 - RNA, 20 nt, synthetic construct
  source 1..20: mol_type = other RNA
gtgaggctgcagctggctgt

SEQ ID NO: 7339 - RNA, 20 nt, synthetic construct
  source 1..20: mol_type = other RNA
gacagccagctgcagcctca

SEQ ID NO: 7340 - RNA, 20 nt, synthetic construct
  source 1..20: mol_type = other RNA
tgcagctggctgtcggcctt

SEQ ID NO: 7341 - RNA, 20 nt, synthetic construct
  source 1..20: mol_type = other RNA
gtcggccttaggctttttgc

SEQ ID NO: 7342 - RNA, 20 nt, synthetic construct
  source 1..20: mol_type = other RNA
cttaggctttttgctggaag

SEQ ID NO: 7343 - RNA, 20 nt, synthetic construct
  source 1..20: mol_type = other RNA
ctcttccagcaaaaagccta

SEQ ID NO: 7344 - RNA, 20 nt, synthetic construct
  source 1..20: mol_type = other RNA
gtaaacaaactgttgccatt

SEQ ID NO: 7345 - RNA, 20 nt, synthetic construct
  source 1..20: mol_type = other RNA
acaaactgttgccattaggt

SEQ ID NO: 7346 - RNA, 20 nt, synthetic construct
  source 1..20: mol_type = other RNA
actgttgccattaggtcggc

SEQ ID NO: 7347 - RNA, 20 nt, synthetic construct
  source 1..20: mol_type = other RNA
acttcttccagccgacctaa

SEQ ID NO: 7348 - RNA, 20 nt, synthetic construct
  source 1..20: mol_type = other RNA
ggaagaagttaagtcctcgc

SEQ ID NO: 7349 - RNA, 20 nt, synthetic construct
  source 1..20: mol_type = other RNA
taaacacaaatacaccagcg

SEQ ID NO: 7350 - RNA, 20 nt, synthetic construct
  source 1..20: mol_type = other RNA
tgtgtttagatgcatcagag

SEQ ID NO: 7351 - RNA, 20 nt, synthetic construct
  source 1..20: mol_type = other RNA
gtgtttagatgcatcagaga

SEQ ID NO: 7352 - RNA, 20 nt, synthetic construct
  source 1..20: mol_type = other RNA
tgtttagatgcatcagagag

SEQ ID NO: 7353 - RNA, 20 nt, synthetic construct
  source 1..20: mol_type = other RNA
tgcatcagagaggggtgaga

SEQ ID NO: 7354 - RNA, 20 nt, synthetic construct
  source 1..20: mol_type = other RNA
gcatcagagaggggtgagat

SEQ ID NO: 7355 - RNA, 20 nt, synthetic construct
  source 1..20: mol_type = other RNA
ataaaaatgaaaaaatgctt

SEQ ID NO: 7356 - RNA, 20 nt, synthetic construct
  source 1..20: mol_type = other RNA
attttttcatttttatttat

SEQ ID NO: 7357 - RNA, 20 nt, synthetic construct
  source 1..20: mol_type = other RNA
tggtattgccacactgaaaa

SEQ ID NO: 7358 - RNA, 20 nt, synthetic construct
  source 1..20: mol_type = other RNA
cacactgaaaaaggaaatta

SEQ ID NO: 7359 - RNA, 20 nt, synthetic construct
  source 1..20: mol_type = other RNA
cgtaatttcctttttcagtg

SEQ ID NO: 7360 - RNA, 20 nt, synthetic construct
  source 1..20: mol_type = other RNA
gaaaaaggaaattacggtaa

SEQ ID NO: 7361 - RNA, 20 nt, synthetic construct
  source 1..20: mol_type = other RNA
gaatgttacagagtcagcac

SEQ ID NO: 7362 - RNA, 20 nt, synthetic construct
  source 1..20: mol_type = other RNA
aatgttacagagtcagcaca

SEQ ID NO: 7363 - RNA, 20 nt, synthetic construct
  source 1..20: mol_type = other RNA
tacagagtcagcacagggaa

SEQ ID NO: 7364 - RNA, 20 nt, synthetic construct
  source 1..20: mol_type = other RNA
tatgacccaaaccacccaac

SEQ ID NO: 7365 - RNA, 20 nt, synthetic construct
  source 1..20: mol_type = other RNA
atgacccaaaccacccaact

SEQ ID NO: 7366 - RNA, 20 nt, synthetic construct
  source 1..20: mol_type = other RNA
accacccaactgggacctgt

SEQ ID NO: 7367 - RNA, 20 nt, synthetic construct
  source 1..20: mol_type = other RNA
caggtcccagttgggtggtt

SEQ ID NO: 7368 - RNA, 20 nt, synthetic construct
  source 1..20: mol_type = other RNA
cccaactgggacctgttggt

SEQ ID NO: 7369 - RNA, 20 nt, synthetic construct
  source 1..20: mol_type = other RNA
accaacaggtcccagttggg

SEQ ID NO: 7370 - RNA, 20 nt, synthetic construct
  source 1..20: mol_type = other RNA
cctaccaacaggtcccagtt

SEQ ID NO: 7371 - RNA, 20 nt, synthetic construct
  source 1..20: mol_type = other RNA
tcctaccaacaggtcccagt

SEQ ID NO: 7372 - RNA, 20 nt, synthetic construct
  source 1..20: mol_type = other RNA
tgttggtaggagaagcttat

SEQ ID NO: 7373 - RNA, 20 nt, synthetic construct
  source 1..20: mol_type = other RNA
gttggtaggagaagcttatt

SEQ ID NO: 7374 - RNA, 20 nt, synthetic construct
  source 1..20: mol_type = other RNA
aataagcttctcctaccaac

SEQ ID NO: 7375 - RNA, 20 nt, synthetic construct
  source 1..20: mol_type = other RNA
tttgaggactactctggtca

SEQ ID NO: 7376 - RNA, 20 nt, synthetic construct
  source 1..20: mol_type = other RNA
aggctttttgaggactactc

SEQ ID NO: 7377 - RNA, 20 nt, synthetic construct
  source 1..20: mol_type = other RNA
gaggagggtcaggctttttg

SEQ ID NO: 7378 - RNA, 20 nt, synthetic construct
  source 1..20: mol_type = other RNA
tgaccctcctccaacatagc

SEQ ID NO: 7379 - RNA, 20 nt, synthetic construct
  source 1..20: mol_type = other RNA
tgctatgttggaggagggtc

SEQ ID NO: 7380 - RNA, 20 nt, synthetic construct
  source 1..20: mol_type = other RNA
tcacctgctatgttggagga

SEQ ID NO: 7381 - RNA, 20 nt, synthetic construct
  source 1..20: mol_type = other RNA
gtcacctgctatgttggagg

SEQ ID NO: 7382 - RNA, 20 nt, synthetic construct
  source 1..20: mol_type = other RNA
aaagtcacctgctatgttgg

SEQ ID NO: 7383 - RNA, 20 nt, synthetic construct
  source 1..20: mol_type = other RNA
ctgaaagtcacctgctatgt

SEQ ID NO: 7384 - RNA, 20 nt, synthetic construct
  source 1..20: mol_type = other RNA
agtgagctggagagatctct

SEQ ID NO: 7385 - RNA, 20 nt, synthetic construct
  source 1..20: mol_type = other RNA
aagtgagctggagagatctc

SEQ ID NO: 7386 - RNA, 20 nt, synthetic construct
  source 1..20: mol_type = other RNA
tctccagctcacttccactt

SEQ ID NO: 7387 - RNA, 20 nt, synthetic construct
  source 1..20: mol_type = other RNA
ccagctcacttccactttgg

SEQ ID NO: 7388 - RNA, 20 nt, synthetic construct
  source 1..20: mol_type = other RNA
cagctcacttccactttgga

SEQ ID NO: 7389 - RNA, 20 nt, synthetic construct
  source 1..20: mol_type = other RNA
cctccaaagtggaagtgagc

SEQ ID NO: 7390 - RNA, 20 nt, synthetic construct
  source 1..20: mol_type = other RNA
tacgtgcattccctccaaag

SEQ ID NO: 7391 - RNA, 20 nt, synthetic construct
  source 1..20: mol_type = other RNA
tgttgatgttcatgttgcag

SEQ ID NO: 7392 - RNA, 20 nt, synthetic construct
  source 1..20: mol_type = other RNA
actgcaacatgaacatcaac

SEQ ID NO: 7393 - RNA, 20 nt, synthetic construct
  source 1..20: mol_type = other RNA
gtttgcagacaaagtattac

SEQ ID NO: 7394 - RNA, 20 nt, synthetic construct
  source 1..20: mol_type = other RNA
tgcagacaaagtattactgg

SEQ ID NO: 7395 - RNA, 20 nt, synthetic construct
  source 1..20: mol_type = other RNA
agacaaagtattactggtgg

SEQ ID NO: 7396 - RNA, 20 nt, synthetic construct
  source 1..20: mol_type = other RNA
caaagtattactggtggagg

SEQ ID NO: 7397 - RNA, 20 nt, synthetic construct
  source 1..20: mol_type = other RNA
gaaagacagctcttcaagac

SEQ ID NO: 7398 - RNA, 20 nt, synthetic construct
  source 1..20: mol_type = other RNA
aagagctgtctttctctccc

SEQ ID NO: 7399 - RNA, 20 nt, synthetic construct
  source 1..20: mol_type = other RNA
agagctgtctttctctccct

SEQ ID NO: 7400 - RNA, 20 nt, synthetic construct
  source 1..20: mol_type = other RNA
agggagatcaagaagtccca

SEQ ID NO: 7401 - RNA, 20 nt, synthetic construct
  source 1..20: mol_type = other RNA
cagggagatcaagaagtccc

SEQ ID NO: 7402 - RNA, 20 nt, synthetic construct
  source 1..20: mol_type = other RNA
tgacaacgaagacgactaca

SEQ ID NO: 7403 - RNA, 20 nt, synthetic construct
  source 1..20: mol_type = other RNA
gtgacaacgaagacgactac

SEQ ID NO: 7404 - RNA, 20 nt, synthetic construct
  source 1..20: mol_type = other RNA
gtcttcgttgtcacactgta

SEQ ID NO: 7405 - RNA, 20 nt, synthetic construct
  source 1..20: mol_type = other RNA
tcttcgttgtcacactgtat

SEQ ID NO: 7406 - RNA, 20 nt, synthetic construct
  source 1..20: mol_type = other RNA
aaactaaagtcaatcagcac

SEQ ID NO: 7407 - RNA, 20 nt, synthetic construct
  source 1..20: mol_type = other RNA
aatcagcactggatttcaag

SEQ ID NO: 7408 - RNA, 20 nt, synthetic construct
  source 1..20: mol_type = other RNA
aagaggtattatgagttccc

SEQ ID NO: 7409 - RNA, 20 nt, synthetic construct
  source 1..20: mol_type = other RNA
gcaccgacttccacagagca

SEQ ID NO: 7410 - RNA, 20 nt, synthetic construct
  source 1..20: mol_type = other RNA
gctctgtggaagtcggtgcc

SEQ ID NO: 7411 - RNA, 20 nt, synthetic construct
  source 1..20: mol_type = other RNA
ttccacagagcaaggcctcc

SEQ ID NO: 7412 - RNA, 20 nt, synthetic construct
  source 1..20: mol_type = other RNA
tccacagagcaaggcctcct

SEQ ID NO: 7413 - RNA, 20 nt, synthetic construct
  source 1..20: mol_type = other RNA
tcccaggaggccttgctctg

SEQ ID NO: 7414 - RNA, 20 nt, synthetic construct
  source 1..20: mol_type = other RNA
tcctgggagccccactcacc

SEQ ID NO: 7415 - RNA, 20 nt, synthetic construct
  source 1..20: mol_type = other RNA
aggtgagtggggctcccagg

SEQ ID NO: 7416 - RNA, 20 nt, synthetic construct
  source 1..20: mol_type = other RNA
gccaggtgagtggggctccc

SEQ ID NO: 7417 - RNA, 20 nt, synthetic construct
  source 1..20: mol_type = other RNA
tcggggaagccaggtgagtg

SEQ ID NO: 7418 - RNA, 20 nt, synthetic construct
  source 1..20: mol_type = other RNA
ttcggggaagccaggtgagt

SEQ ID NO: 7419 - RNA, 20 nt, synthetic construct
  source 1..20: mol_type = other RNA
cttcggggaagccaggtgag

SEQ ID NO: 7420 - RNA, 20 nt, synthetic construct
  source 1..20: mol_type = other RNA
ttgggacggtaggctgccgc

SEQ ID NO: 7421 - RNA, 20 nt, synthetic construct
  source 1..20: mol_type = other RNA
ccgtcccaaacagcagccta

SEQ ID NO: 7422 - RNA, 20 nt, synthetic construct
  source 1..20: mol_type = other RNA
aggctgctgtttgggacggt

SEQ ID NO: 7423 - RNA, 20 nt, synthetic construct
  source 1..20: mol_type = other RNA
ccataggctgctgtttggga

SEQ ID NO: 7424 - RNA, 20 nt, synthetic construct
  source 1..20: mol_type = other RNA
gcacccataggctgctgttt

SEQ ID NO: 7425 - RNA, 20 nt, synthetic construct
  source 1..20: mol_type = other RNA
agcacccataggctgctgtt

SEQ ID NO: 7426 - RNA, 20 nt, synthetic construct
  source 1..20: mol_type = other RNA
tacttggatagagcacccat

SEQ ID NO: 7427 - RNA, 20 nt, synthetic construct
  source 1..20: mol_type = other RNA
tctcttaacttgtgggtact

SEQ ID NO: 7428 - RNA, 20 nt, synthetic construct
  source 1..20: mol_type = other RNA
ggggctatctcttaacttgt

SEQ ID NO: 7429 - RNA, 20 nt, synthetic construct
  source 1..20: mol_type = other RNA
aggggctatctcttaacttg

SEQ ID NO: 7430 - RNA, 20 nt, synthetic construct
  source 1..20: mol_type = other RNA
gcgggggcgtggaggggaag

SEQ ID NO: 7431 - RNA, 20 nt, synthetic construct
  source 1..20: mol_type = other RNA
tgcgggggcgtggaggggaa

SEQ ID NO: 7432 - RNA, 20 nt, synthetic construct
  source 1..20: mol_type = other RNA
gtgcgggggcgtggagggga

SEQ ID NO: 7433 - RNA, 20 nt, synthetic construct
  source 1..20: mol_type = other RNA
tggggtgcgggggcgtggag

SEQ ID NO: 7434 - RNA, 20 nt, synthetic construct
  source 1..20: mol_type = other RNA
ctggggtgcgggggcgtgga

SEQ ID NO: 7435 - RNA, 20 nt, synthetic construct
  source 1..20: mol_type = other RNA
actggggtgcgggggcgtgg

SEQ ID NO: 7436 - RNA, 20 nt, synthetic construct
  source 1..20: mol_type = other RNA
ctgactggggtgcgggggcg

SEQ ID NO: 7437 - RNA, 20 nt, synthetic construct
  source 1..20: mol_type = other RNA
cccgcaccccagtcagcccc

SEQ ID NO: 7438 - RNA, 20 nt, synthetic construct
  source 1..20: mol_type = other RNA
tggggctgactggggtgcgg

SEQ ID NO: 7439 - RNA, 20 nt, synthetic construct
  source 1..20: mol_type = other RNA
ctggggctgactggggtgcg

SEQ ID NO: 7440 - RNA, 20 nt, synthetic construct
  source 1..20: mol_type = other RNA
cctggggctgactggggtgc

SEQ ID NO: 7441 - RNA, 20 nt, synthetic construct
  source 1..20: mol_type = other RNA
gcctggggctgactggggtg

SEQ ID NO: 7442 - RNA, 20 nt, synthetic construct
  source 1..20: mol_type = other RNA
ggtaggcctggggctgactg

SEQ ID NO: 7443 - RNA, 20 nt, synthetic construct
  source 1..20: mol_type = other RNA
aggtaggcctggggctgact

SEQ ID NO: 7444 - RNA, 20 nt, synthetic construct
  source 1..20: mol_type = other RNA
aaggtaggcctggggctgac

SEQ ID NO: 7445 - RNA, 20 nt, synthetic construct
  source 1..20: mol_type = other RNA
ggaaacgcaaggtaggcctg

SEQ ID NO: 7446 - RNA, 20 nt, synthetic construct
  source 1..20: mol_type = other RNA
gcctaccttgcgtttcctct

SEQ ID NO: 7447 - RNA, 20 nt, synthetic construct
  source 1..20: mol_type = other RNA
gaggaaacgcaaggtaggcc

SEQ ID NO: 7448 - RNA, 20 nt, synthetic construct
  source 1..20: mol_type = other RNA
tccaagaggaaacgcaaggt

SEQ ID NO: 7449 - RNA, 20 nt, synthetic construct
  source 1..20: mol_type = other RNA
ttgcgtttcctcttggattt

SEQ ID NO: 7450 - RNA, 20 nt, synthetic construct
  source 1..20: mol_type = other RNA
aaaatccaagaggaaacgca

SEQ ID NO: 7451 - RNA, 20 nt, synthetic construct
  source 1..20: mol_type = other RNA
aggctttgccaaaatccaag

SEQ ID NO: 7452 - RNA, 20 nt, synthetic construct
  source 1..20: mol_type = other RNA
tttggcaaagccttttctgc

SEQ ID NO: 7453 - RNA, 20 nt, synthetic construct
  source 1..20: mol_type = other RNA
cttttctgcaggtgtgtccg

SEQ ID NO: 7454 - RNA, 20 nt, synthetic construct
  source 1..20: mol_type = other RNA
ctcggacacacctgcagaaa

SEQ ID NO: 7455 - RNA, 20 nt, synthetic construct
  source 1..20: mol_type = other RNA
ctgcaggtgtgtccgaggtg

SEQ ID NO: 7456 - RNA, 20 nt, synthetic construct
  source 1..20: mol_type = other RNA
aggtgtgtccgaggtgtggc

SEQ ID NO: 7457 - RNA, 20 nt, synthetic construct
  source 1..20: mol_type = other RNA
ggtgtgtccgaggtgtggct

SEQ ID NO: 7458 - RNA, 20 nt, synthetic construct
  source 1..20: mol_type = other RNA
gtgtccgaggtgtggctggg

SEQ ID NO: 7459 - RNA, 20 nt, synthetic construct
  source 1..20: mol_type = other RNA
cgcaccgcccagccacacct

SEQ ID NO: 7460 - RNA, 20 nt, synthetic construct
  source 1..20: mol_type = other RNA
cggtgcgctctcagagtcct

SEQ ID NO: 7461 - RNA, 20 nt, synthetic construct
  source 1..20: mol_type = other RNA
tgcgctctcagagtccttgg

SEQ ID NO: 7462 - RNA, 20 nt, synthetic construct
  source 1..20: mol_type = other RNA
ctctcagagtccttggtggc

SEQ ID NO: 7463 - RNA, 20 nt, synthetic construct
  source 1..20: mol_type = other RNA
tctcagagtccttggtggca

SEQ ID NO: 7464 - RNA, 20 nt, synthetic construct
  source 1..20: mol_type = other RNA
ctcagagtccttggtggcag

SEQ ID NO: 7465 - RNA, 20 nt, synthetic construct
  source 1..20: mol_type = other RNA
attgagcgcccctgccacca

SEQ ID NO: 7466 - RNA, 20 nt, synthetic construct
  source 1..20: mol_type = other RNA
gcaggggcgctcaatacccc

SEQ ID NO: 7467 - RNA, 20 nt, synthetic construct
  source 1..20: mol_type = other RNA
cgctcaatacccctggctcc

SEQ ID NO: 7468 - RNA, 20 nt, synthetic construct
  source 1..20: mol_type = other RNA
gctcaatacccctggctcct

SEQ ID NO: 7469 - RNA, 20 nt, synthetic construct
  source 1..20: mol_type = other RNA
ctcaatacccctggctcctg

SEQ ID NO: 7470 - RNA, 20 nt, synthetic construct
  source 1..20: mol_type = other RNA
atacccctggctcctggggc

SEQ ID NO: 7471 - RNA, 20 nt, synthetic construct
  source 1..20: mol_type = other RNA
ggctcctggggcaggtgttc

SEQ ID NO: 7472 - RNA, 20 nt, synthetic construct
  source 1..20: mol_type = other RNA
aacacctgccccaggagcca

SEQ ID NO: 7473 - RNA, 20 nt, synthetic construct
  source 1..20: mol_type = other RNA
gaacacctgccccaggagcc

SEQ ID NO: 7474 - RNA, 20 nt, synthetic construct
  source 1..20: mol_type = other RNA
gggcaggtgttctgggatcc

SEQ ID NO: 7475 - RNA, 20 nt, synthetic construct
  source 1..20: mol_type = other RNA
gatcccagaacacctgcccc

SEQ ID NO: 7476 - RNA, 20 nt, synthetic construct
  source 1..20: mol_type = other RNA
ggtgttctgggatcctggac

SEQ ID NO: 7477 - RNA, 20 nt, synthetic construct
  source 1..20: mol_type = other RNA
gttctgggatcctggacagg

SEQ ID NO: 7478 - RNA, 20 nt, synthetic construct
  source 1..20: mol_type = other RNA
ttctgggatcctggacagga

SEQ ID NO: 7479 - RNA, 20 nt, synthetic construct
  source 1..20: mol_type = other RNA
ggatcctggacaggagggtc

SEQ ID NO: 7480 - RNA, 20 nt, synthetic construct
  source 1..20: mol_type = other RNA
tcgacctgaccctcctgtcc

SEQ ID NO: 7481 - RNA, 20 nt, synthetic construct
  source 1..20: mol_type = other RNA
tgatgagatcaggtctctct

SEQ ID NO: 7482 - RNA, 20 nt, synthetic construct
  source 1..20: mol_type = other RNA
gtgatgagatcaggtctctc

SEQ ID NO: 7483 - RNA, 20 nt, synthetic construct
  source 1..20: mol_type = other RNA
atctcatcactgtcctttag

SEQ ID NO: 7484 - RNA, 20 nt, synthetic construct
  source 1..20: mol_type = other RNA
tctcatcactgtcctttaga

SEQ ID NO: 7485 - RNA, 20 nt, synthetic construct
  source 1..20: mol_type = other RNA
ctcatcactgtcctttagag

SEQ ID NO: 7486 - RNA, 20 nt, synthetic construct
  source 1..20: mol_type = other RNA
cgaacttctctcccctctaa

SEQ ID NO: 7487 - RNA, 20 nt, synthetic construct
  source 1..20: mol_type = other RNA
gaggggagagaagttcgttc

SEQ ID NO: 7488 - RNA, 20 nt, synthetic construct
  source 1..20: mol_type = other RNA
gagaagttcgttccggccaa

SEQ ID NO: 7489 - RNA, 20 nt, synthetic construct
  source 1..20: mol_type = other RNA
agaagttcgttccggccaaa

SEQ ID NO: 7490 - RNA, 20 nt, synthetic construct
  source 1..20: mol_type = other RNA
gaagttcgttccggccaaag

SEQ ID NO: 7491 - RNA, 20 nt, synthetic construct
  source 1..20: mol_type = other RNA
acacactggtcccctttggc

SEQ ID NO: 7492 - RNA, 20 nt, synthetic construct
  source 1..20: mol_type = other RNA
ttctacacactggtcccctt

SEQ ID NO: 7493 - RNA, 20 nt, synthetic construct
  source 1..20: mol_type = other RNA
ggaggagcagttctacacac

SEQ ID NO: 7494 - RNA, 20 nt, synthetic construct
  source 1..20: mol_type = other RNA
gaactgctcctccagctcct

SEQ ID NO: 7495 - RNA, 20 nt, synthetic construct
  source 1..20: mol_type = other RNA
cagctccttggcgatgtcac

SEQ ID NO: 7496 - RNA, 20 nt, synthetic construct
  source 1..20: mol_type = other RNA
tgacatcgccaaggagctgg

SEQ ID NO: 7497 - RNA, 20 nt, synthetic construct
  source 1..20: mol_type = other RNA
ctccttggcgatgtcactgg

SEQ ID NO: 7498 - RNA, 20 nt, synthetic construct
  source 1..20: mol_type = other RNA
cagtgacatcgccaaggagc

SEQ ID NO: 7499 - RNA, 20 nt, synthetic construct
  source 1..20: mol_type = other RNA
ggcgatgtcactggtggtcc

SEQ ID NO: 7500 - RNA, 20 nt, synthetic construct
  source 1..20: mol_type = other RNA
gaccaccagtgacatcgcca

SEQ ID NO: 7501 - RNA, 20 nt, synthetic construct
  source 1..20: mol_type = other RNA
actggtggtcctggcgttga

SEQ ID NO: 7502 - RNA, 20 nt, synthetic construct
  source 1..20: mol_type = other RNA
ctggcgttgatggagcctac

SEQ ID NO: 7503 - RNA, 20 nt, synthetic construct
  source 1..20: mol_type = other RNA
tggcgttgatggagcctaca

SEQ ID NO: 7504 - RNA, 20 nt, synthetic construct
  source 1..20: mol_type = other RNA
ggcgttgatggagcctacag

SEQ ID NO: 7505 - RNA, 20 nt, synthetic construct
  source 1..20: mol_type = other RNA
ctgtaggctccatcaacgcc

SEQ ID NO: 7506 - RNA, 20 nt, synthetic construct
  source 1..20: mol_type = other RNA
atggagcctacaggggccct

SEQ ID NO: 7507 - RNA, 20 nt, synthetic construct
  source 1..20: mol_type = other RNA
agtggtcctagggcccctgt

SEQ ID NO: 7508 - RNA, 20 nt, synthetic construct
  source 1..20: mol_type = other RNA
cctaggaccactgcccccgt

SEQ ID NO: 7509 - RNA, 20 nt, synthetic construct
  source 1..20: mol_type = other RNA
caacgggggcagtggtccta

SEQ ID NO: 7510 - RNA, 20 nt, synthetic construct
  source 1..20: mol_type = other RNA
ccaacgggggcagtggtcct

SEQ ID NO: 7511 - RNA, 20 nt, synthetic construct
  source 1..20: mol_type = other RNA
accactgcccccgttggcag

SEQ ID NO: 7512 - RNA, 20 nt, synthetic construct
  source 1..20: mol_type = other RNA
gccgctgccaacgggggcag

SEQ ID NO: 7513 - RNA, 20 nt, synthetic construct
  source 1..20: mol_type = other RNA
aaggaggccgctgccaacgg

SEQ ID NO: 7514 - RNA, 20 nt, synthetic construct
  source 1..20: mol_type = other RNA
gaaggaggccgctgccaacg

SEQ ID NO: 7515 - RNA, 20 nt, synthetic construct
  source 1..20: mol_type = other RNA
tgaaggaggccgctgccaac

SEQ ID NO: 7516 - RNA, 20 nt, synthetic construct
  source 1..20: mol_type = other RNA
ctgaaggaggccgctgccaa

SEQ ID NO: 7517 - RNA, 20 nt, synthetic construct
  source 1..20: mol_type = other RNA
cttcagcctctgatcattcc

SEQ ID NO: 7518 - RNA, 20 nt, synthetic construct
  source 1..20: mol_type = other RNA
gaatgatcagaggctgaagg

SEQ ID NO: 7519 - RNA, 20 nt, synthetic construct
  source 1..20: mol_type = other RNA
cagcctctgatcattcccgg

SEQ ID NO: 7520 - RNA, 20 nt, synthetic construct
  source 1..20: mol_type = other RNA
cgggaatgatcagaggctga

SEQ ID NO: 7521 - RNA, 20 nt, synthetic construct
  source 1..20: mol_type = other RNA
cctctgatcattcccggagg

SEQ ID NO: 7522 - RNA, 20 nt, synthetic construct
  source 1..20: mol_type = other RNA
cctcctccgggaatgatcag

SEQ ID NO: 7523 - RNA, 20 nt, synthetic construct
  source 1..20: mol_type = other RNA
atcattcccggaggaggcag

SEQ ID NO: 7524 - RNA, 20 nt, synthetic construct
  source 1..20: mol_type = other RNA
ggaggaggcagaggcagcca

SEQ ID NO: 7525 - RNA, 20 nt, synthetic construct
  source 1..20: mol_type = other RNA
tggctgcctctgcctcctcc

SEQ ID NO: 7526 - RNA, 20 nt, synthetic construct
  source 1..20: mol_type = other RNA
gtggctgcctctgcctcctc

SEQ ID NO: 7527 - RNA, 20 nt, synthetic construct
  source 1..20: mol_type = other RNA
ggcagccacggtctgtgctt

SEQ ID NO: 7528 - RNA, 20 nt, synthetic construct
  source 1..20: mol_type = other RNA
acggtctgtgctttggacag

SEQ ID NO: 7529 - RNA, 20 nt, synthetic construct
  source 1..20: mol_type = other RNA
cggtctgtgctttggacaga

SEQ ID NO: 7530 - RNA, 20 nt, synthetic construct
  source 1..20: mol_type = other RNA
tctgtccaaagcacagaccg

SEQ ID NO: 7531 - RNA, 20 nt, synthetic construct
  source 1..20: mol_type = other RNA
cagagggtactcctcctgct

SEQ ID NO: 7532 - RNA, 20 nt, synthetic construct
  source 1..20: mol_type = other RNA
actcctcctgctcggactcc

SEQ ID NO: 7533 - RNA, 20 nt, synthetic construct
  source 1..20: mol_type = other RNA
ctcctgctcggactccaggt

SEQ ID NO: 7534 - RNA, 20 nt, synthetic construct
  source 1..20: mol_type = other RNA
cgacctggagtccgagcagg

SEQ ID NO: 7535 - RNA, 20 nt, synthetic construct
  source 1..20: mol_type = other RNA
ctccgacctggagtccgagc

SEQ ID NO: 7536 - RNA, 20 nt, synthetic construct
  source 1..20: mol_type = other RNA
ggactccaggtcggagtccg

SEQ ID NO: 7537 - RNA, 20 nt, synthetic construct
  source 1..20: mol_type = other RNA
ctccaggtcggagtccgagg

SEQ ID NO: 7538 - RNA, 20 nt, synthetic construct
  source 1..20: mol_type = other RNA
caggtcggagtccgaggagg

SEQ ID NO: 7539 - RNA, 20 nt, synthetic construct
  source 1..20: mol_type = other RNA
ctcctcctcggactccgacc

SEQ ID NO: 7540 - RNA, 20 nt, synthetic construct
  source 1..20: mol_type = other RNA
gtcatcttcatcctcctcct

SEQ ID NO: 7541 - RNA, 20 nt, synthetic construct
  source 1..20: mol_type = other RNA
ctctgtctcaatgaactcct

SEQ ID NO: 7542 - RNA, 20 nt, synthetic construct
  source 1..20: mol_type = other RNA
ctcaatgaactccttggatt

SEQ ID NO: 7543 - RNA, 20 nt, synthetic construct
  source 1..20: mol_type = other RNA
tcaatgaactccttggattt

SEQ ID NO: 7544 - RNA, 20 nt, synthetic construct
  source 1..20: mol_type = other RNA
caatgaactccttggatttg

SEQ ID NO: 7545 - RNA, 20 nt, synthetic construct
  source 1..20: mol_type = other RNA
caggatcgtccccaaatcca

SEQ ID NO: 7546 - RNA, 20 nt, synthetic construct
  source 1..20: mol_type = other RNA
tcctgcttagcccccgcgtg

SEQ ID NO: 7547 - RNA, 20 nt, synthetic construct
  source 1..20: mol_type = other RNA
gccgcacgcgggggctaagc

SEQ ID NO: 7548 - RNA, 20 nt, synthetic construct
  source 1..20: mol_type = other RNA
ccgcgtgcggcgcttctcgc

SEQ ID NO: 7549 - RNA, 20 nt, synthetic construct
  source 1..20: mol_type = other RNA
gcgagaagcgccgcacgcgg

SEQ ID NO: 7550 - RNA, 20 nt, synthetic construct
  source 1..20: mol_type = other RNA
tgcgagaagcgccgcacgcg

SEQ ID NO: 7551 - RNA, 20 nt, synthetic construct
  source 1..20: mol_type = other RNA
ctgcgagaagcgccgcacgc

SEQ ID NO: 7552 - RNA, 20 nt, synthetic construct
  source 1..20: mol_type = other RNA
cctgcgagaagcgccgcacg

SEQ ID NO: 7553 - RNA, 20 nt, synthetic construct
  source 1..20: mol_type = other RNA
gcggcgcttctcgcaggtca

SEQ ID NO: 7554 - RNA, 20 nt, synthetic construct
  source 1..20: mol_type = other RNA
gcgcttctcgcaggtcacgg

SEQ ID NO: 7555 - RNA, 20 nt, synthetic construct
  source 1..20: mol_type = other RNA
cggaggagcgcagctccttg

SEQ ID NO: 7556 - RNA, 20 nt, synthetic construct
  source 1..20: mol_type = other RNA
aggagcgcagctccttgcgg

SEQ ID NO: 7557 - RNA, 20 nt, synthetic construct
  source 1..20: mol_type = other RNA
caacagagcgagccaccgca

SEQ ID NO: 7558 - RNA, 20 nt, synthetic construct
  source 1..20: mol_type = other RNA
gctcgctctgttgttgccac

SEQ ID NO: 7559 - RNA, 20 nt, synthetic construct
  source 1..20: mol_type = other RNA
ctcgctctgttgttgccaca

SEQ ID NO: 7560 - RNA, 20 nt, synthetic construct
  source 1..20: mol_type = other RNA
tctgttgttgccacagggcc

SEQ ID NO: 7561 - RNA, 20 nt, synthetic construct
  source 1..20: mol_type = other RNA
gttgccacagggcctggttt

SEQ ID NO: 7562 - RNA, 20 nt, synthetic construct
  source 1..20: mol_type = other RNA
gccacagggcctggttttgg

SEQ ID NO: 7563 - RNA, 20 nt, synthetic construct
  source 1..20: mol_type = other RNA
ccacagggcctggttttggt

SEQ ID NO: 7564 - RNA, 20 nt, synthetic construct
  source 1..20: mol_type = other RNA
cccaccaaaaccaggccctg

SEQ ID NO: 7565 - RNA, 20 nt, synthetic construct
  source 1..20: mol_type = other RNA
ggcctggttttggtgggctc

SEQ ID NO: 7566 - RNA, 20 nt, synthetic construct
  source 1..20: mol_type = other RNA
gcctggttttggtgggctcc

SEQ ID NO: 7567 - RNA, 20 nt, synthetic construct
  source 1..20: mol_type = other RNA
cctggttttggtgggctccg

SEQ ID NO: 7568 - RNA, 20 nt, synthetic construct
  source 1..20: mol_type = other RNA
ctggttttggtgggctccgg

SEQ ID NO: 7569 - RNA, 20 nt, synthetic construct
  source 1..20: mol_type = other RNA
tggttttggtgggctccggg

SEQ ID NO: 7570 - RNA, 20 nt, synthetic construct
  source 1..20: mol_type = other RNA
ccccggagcccaccaaaacc

SEQ ID NO: 7571 - RNA, 20 nt, synthetic construct
  source 1..20: mol_type = other RNA
gacgagcgtggtggtccccc

SEQ ID NO: 7572 - RNA, 20 nt, synthetic construct
  source 1..20: mol_type = other RNA
cgcgctggggacgagcgtgg

SEQ ID NO: 7573 - RNA, 20 nt, synthetic construct
  source 1..20: mol_type = other RNA
gctcgtccccagcgcgtccg

SEQ ID NO: 7574 - RNA, 20 nt, synthetic construct
  source 1..20: mol_type = other RNA
ggacgcgctggggacgagcg

SEQ ID NO: 7575 - RNA, 20 nt, synthetic construct
  source 1..20: mol_type = other RNA
ccccagcgcgtccgcggccg

SEQ ID NO: 7576 - RNA, 20 nt, synthetic construct
  source 1..20: mol_type = other RNA
cccagcgcgtccgcggccgc

SEQ ID NO: 7577 - RNA, 20 nt, synthetic construct
  source 1..20: mol_type = other RNA
ccgcggccgcggacgcgctg

SEQ ID NO: 7578 - RNA, 20 nt, synthetic construct
  source 1..20: mol_type = other RNA
cccgcggccgcggacgcgct

SEQ ID NO: 7579 - RNA, 20 nt, synthetic construct
  source 1..20: mol_type = other RNA
gcccgcggccgcggacgcgc

SEQ ID NO: 7580 - RNA, 20 nt, synthetic construct
  source 1..20: mol_type = other RNA
gtccgcggccgcgggctcct

SEQ ID NO: 7581 - RNA, 20 nt, synthetic construct
  source 1..20: mol_type = other RNA
tccgcggccgcgggctcctc

SEQ ID NO: 7582 - RNA, 20 nt, synthetic construct
  source 1..20: mol_type = other RNA
cggccgcgggctcctcgggc

SEQ ID NO: 7583 - RNA, 20 nt, synthetic construct
  source 1..20: mol_type = other RNA
gcccgaggagcccgcggccg

SEQ ID NO: 7584 - RNA, 20 nt, synthetic construct
  source 1..20: mol_type = other RNA
ccgcgggctcctcgggccgg

SEQ ID NO: 7585 - RNA, 20 nt, synthetic construct
  source 1..20: mol_type = other RNA
ccaccggcccgaggagcccg

SEQ ID NO: 7586 - RNA, 20 nt, synthetic construct
  source 1..20: mol_type = other RNA
ctcctcgggccggtggcagt

SEQ ID NO: 7587 - RNA, 20 nt, synthetic construct
  source 1..20: mol_type = other RNA
cgccaactgccaccggcccg

SEQ ID NO: 7588 - RNA, 20 nt, synthetic construct
  source 1..20: mol_type = other RNA
gtggcagttggcgccgtccc

SEQ ID NO: 7589 - RNA, 20 nt, synthetic construct
  source 1..20: mol_type = other RNA
gggacggcgccaactgccac

SEQ ID NO: 7590 - RNA, 20 nt, synthetic construct
  source 1..20: mol_type = other RNA
gttggcgccgtccccggctg

SEQ ID NO: 7591 - RNA, 20 nt, synthetic construct
  source 1..20: mol_type = other RNA
gtccccggctgaggtcctct

SEQ ID NO: 7592 - RNA, 20 nt, synthetic construct
  source 1..20: mol_type = other RNA
gagaggacctcagccgggga

SEQ ID NO: 7593 - RNA, 20 nt, synthetic construct
  source 1..20: mol_type = other RNA
caccgagaggacctcagccg

SEQ ID NO: 7594 - RNA, 20 nt, synthetic construct
  source 1..20: mol_type = other RNA
gcaccgagaggacctcagcc

SEQ ID NO: 7595 - RNA, 20 nt, synthetic construct
  source 1..20: mol_type = other RNA
cgcaccgagaggacctcagc

SEQ ID NO: 7596 - RNA, 20 nt, synthetic construct
  source 1..20: mol_type = other RNA
ggtcctctcggtgcgcctgg

SEQ ID NO: 7597 - RNA, 20 nt, synthetic construct
  source 1..20: mol_type = other RNA
gtcctctcggtgcgcctggt

SEQ ID NO: 7598 - RNA, 20 nt, synthetic construct
  source 1..20: mol_type = other RNA
agcccaccaggcgcaccgag

SEQ ID NO: 7599 - RNA, 20 nt, synthetic construct
  source 1..20: mol_type = other RNA
cctggtgggcttcttgcccg

SEQ ID NO: 7600 - RNA, 20 nt, synthetic construct
  source 1..20: mol_type = other RNA
ccgcgggcaagaagcccacc

SEQ ID NO: 7601 - RNA, 20 nt, synthetic construct
  source 1..20: mol_type = other RNA
gcttcttgcccgcggacctc

SEQ ID NO: 7602 - RNA, 20 nt, synthetic construct
  source 1..20: mol_type = other RNA
cttcttgcccgcggacctcc

SEQ ID NO: 7603 - RNA, 20 nt, synthetic construct
  source 1..20: mol_type = other RNA
ttgcccgcggacctccgggc

SEQ ID NO: 7604 - RNA, 20 nt, synthetic construct
  source 1..20: mol_type = other RNA
cgcggacctccgggcaggcg

SEQ ID NO: 7605 - RNA, 20 nt, synthetic construct
  source 1..20: mol_type = other RNA
gcggacctccgggcaggcgc

SEQ ID NO: 7606 - RNA, 20 nt, synthetic construct
  source 1..20: mol_type = other RNA
gcgcctgcccggaggtccgc

SEQ ID NO: 7607 - RNA, 20 nt, synthetic construct
  source 1..20: mol_type = other RNA
cgcgcctgcccggaggtccg

SEQ ID NO: 7608 - RNA, 20 nt, synthetic construct
  source 1..20: mol_type = other RNA
acgcgcccgcgcctgcccgg

SEQ ID NO: 7609 - RNA, 20 nt, synthetic construct
  source 1..20: mol_type = other RNA
agaacgcgcccgcgcctgcc

SEQ ID NO: 7610 - RNA, 20 nt, synthetic construct
  source 1..20: mol_type = other RNA
aggcgcgggcgcgttctccg

SEQ ID NO: 7611 - RNA, 20 nt, synthetic construct
  source 1..20: mol_type = other RNA
ggcgcgggcgcgttctccgc

SEQ ID NO: 7612 - RNA, 20 nt, synthetic construct
  source 1..20: mol_type = other RNA
cgcgttctccgcgggcgcac

SEQ ID NO: 7613 - RNA, 20 nt, synthetic construct
  source 1..20: mol_type = other RNA
gcgttctccgcgggcgcaca

SEQ ID NO: 7614 - RNA, 20 nt, synthetic construct
  source 1..20: mol_type = other RNA
cgcgggcgcacagggcactg

SEQ ID NO: 7615 - RNA, 20 nt, synthetic construct
  source 1..20: mol_type = other RNA
gcgggcgcacagggcactgc

SEQ ID NO: 7616 - RNA, 20 nt, synthetic construct
  source 1..20: mol_type = other RNA
ggcgcacagggcactgcggg

SEQ ID NO: 7617 - RNA, 20 nt, synthetic construct
  source 1..20: mol_type = other RNA
gcacagggcactgcgggtgg

SEQ ID NO: 7618 - RNA, 20 nt, synthetic construct
  source 1..20: mol_type = other RNA
cacagggcactgcgggtggc

SEQ ID NO: 7619 - RNA, 20 nt, synthetic construct
  source 1..20: mol_type = other RNA
acagggcactgcgggtggcg

SEQ ID NO: 7620 - RNA, 20 nt, synthetic construct
  source 1..20: mol_type = other RNA
gggcactgcgggtggcgggg

SEQ ID NO: 7621 - RNA, 20 nt, synthetic construct
  source 1..20: mol_type = other RNA
ggcggctgcgctcaccgcca

SEQ ID NO: 7622 - RNA, 20 nt, synthetic construct
  source 1..20: mol_type = other RNA
tgcgctcaccgccacggcca

SEQ ID NO: 7623 - RNA, 20 nt, synthetic construct
  source 1..20: mol_type = other RNA
caccgccacggccacggccg

SEQ ID NO: 7624 - RNA, 20 nt, synthetic construct
  source 1..20: mol_type = other RNA
accgccacggccacggccgc

SEQ ID NO: 7625 - RNA, 20 nt, synthetic construct
  source 1..20: mol_type = other RNA
gccacggccacggccgcggg

SEQ ID NO: 7626 - RNA, 20 nt, synthetic construct
  source 1..20: mol_type = other RNA
ccacggccacggccgcgggc

SEQ ID NO: 7627 - RNA, 20 nt, synthetic construct
  source 1..20: mol_type = other RNA
cacggccacggccgcgggcg

SEQ ID NO: 7628 - RNA, 20 nt, synthetic construct
  source 1..20: mol_type = other RNA
gcccgcggccgtggccgtgg

SEQ ID NO: 7629 - RNA, 20 nt, synthetic construct
  source 1..20: mol_type = other RNA
cccgcccgcggccgtggccg

SEQ ID NO: 7630 - RNA, 20 nt, synthetic construct
  source 1..20: mol_type = other RNA
gaagtccccgcccgcggccg

SEQ ID NO: 7631 - RNA, 20 nt, synthetic construct
  source 1..20: mol_type = other RNA
gaagcagaagtccccgcccg

SEQ ID NO: 7632 - RNA, 20 nt, synthetic construct
  source 1..20: mol_type = other RNA
tgcttcacgcctttactccc

SEQ ID NO: 7633 - RNA, 20 nt, synthetic construct
  source 1..20: mol_type = other RNA
gcttcacgcctttactccca

SEQ ID NO: 7634 - RNA, 20 nt, synthetic construct
  source 1..20: mol_type = other RNA
cttcacgcctttactcccag

SEQ ID NO: 7635 - RNA, 20 nt, synthetic construct
  source 1..20: mol_type = other RNA
tttactcccaggggccttgt

SEQ ID NO: 7636 - RNA, 20 nt, synthetic construct
  source 1..20: mol_type = other RNA
aacaaggcccctgggagtaa

SEQ ID NO: 7637 - RNA, 20 nt, synthetic construct
  source 1..20: mol_type = other RNA
ggggccttgttggctgtcct

SEQ ID NO: 7638 - RNA, 20 nt, synthetic construct
  source 1..20: mol_type = other RNA
ggacagccaacaaggcccct

SEQ ID NO: 7639 - RNA, 20 nt, synthetic construct
  source 1..20: mol_type = other RNA
aggacagccaacaaggcccc

SEQ ID NO: 7640 - RNA, 20 nt, synthetic construct
  source 1..20: mol_type = other RNA
aaggccaaggacagccaaca

SEQ ID NO: 7641 - RNA, 20 nt, synthetic construct
  source 1..20: mol_type = other RNA
gcaaggaggagcaaaggcca

SEQ ID NO: 7642 - RNA, 20 nt, synthetic construct
  source 1..20: mol_type = other RNA
gcacttgcaaggaggagcaa

SEQ ID NO: 7643 - RNA, 20 nt, synthetic construct
  source 1..20: mol_type = other RNA
gatcaagagcacttgcaagg

SEQ ID NO: 7644 - RNA, 20 nt, synthetic construct
  source 1..20: mol_type = other RNA
ggagatcaagagcacttgca

SEQ ID NO: 7645 - RNA, 20 nt, synthetic construct
  source 1..20: mol_type = other RNA
tcttgatctccttctctctc

SEQ ID NO: 7646 - RNA, 20 nt, synthetic construct
  source 1..20: mol_type = other RNA
gatctccttctctctcaggc

SEQ ID NO: 7647 - RNA, 20 nt, synthetic construct
  source 1..20: mol_type = other RNA
atctccttctctctcaggct

SEQ ID NO: 7648 - RNA, 20 nt, synthetic construct
  source 1..20: mol_type = other RNA
ccttctctctcaggctgggc

SEQ ID NO: 7649 - RNA, 20 nt, synthetic construct
  source 1..20: mol_type = other RNA
ccagcccagcctgagagaga

SEQ ID NO: 7650 - RNA, 20 nt, synthetic construct
  source 1..20: mol_type = other RNA
caggctgggctggcaaacgt

SEQ ID NO: 7651 - RNA, 20 nt, synthetic construct
  source 1..20: mol_type = other RNA
aggctgggctggcaaacgtc

SEQ ID NO: 7652 - RNA, 20 nt, synthetic construct
  source 1..20: mol_type = other RNA
ggctgggctggcaaacgtcg

SEQ ID NO: 7653 - RNA, 20 nt, synthetic construct
  source 1..20: mol_type = other RNA
cggggactttcccacagtcc

SEQ ID NO: 7654 - RNA, 20 nt, synthetic construct
  source 1..20: mol_type = other RNA
aagaggacgtccaggactgt

SEQ ID NO: 7655 - RNA, 20 nt, synthetic construct
  source 1..20: mol_type = other RNA
aaagaggacgtccaggactg

SEQ ID NO: 7656 - RNA, 20 nt, synthetic construct
  source 1..20: mol_type = other RNA
tcctggacgtcctctttcac

SEQ ID NO: 7657 - RNA, 20 nt, synthetic construct
  source 1..20: mol_type = other RNA
cctggacgtcctctttcacc

SEQ ID NO: 7658 - RNA, 20 nt, synthetic construct
  source 1..20: mol_type = other RNA
cccggtgaaagaggacgtcc

SEQ ID NO: 7659 - RNA, 20 nt, synthetic construct
  source 1..20: mol_type = other RNA
gtactacaacccggtgaaag

SEQ ID NO: 7660 - RNA, 20 nt, synthetic construct
  source 1..20: mol_type = other RNA
gagcaatcagtactacaacc

SEQ ID NO: 7661 - RNA, 20 nt, synthetic construct
  source 1..20: mol_type = other RNA
actgattgctctctgacccg

SEQ ID NO: 7662 - RNA, 20 nt, synthetic construct
  source 1..20: mol_type = other RNA
ctgacccgtggctttcattt

SEQ ID NO: 7663 - RNA, 20 nt, synthetic construct
  source 1..20: mol_type = other RNA
tgatccaaaatgaaagccac

SEQ ID NO: 7664 - RNA, 20 nt, synthetic construct
  source 1..20: mol_type = other RNA
ctgatccaaaatgaaagcca

SEQ ID NO: 7665 - RNA, 20 nt, synthetic construct
  source 1..20: mol_type = other RNA
ctttcattttggatcagaat

SEQ ID NO: 7666 - RNA, 20 nt, synthetic construct
  source 1..20: mol_type = other RNA
tcattttggatcagaatagg

SEQ ID NO: 7667 - RNA, 20 nt, synthetic construct
  source 1..20: mol_type = other RNA
ggatcagaataggaggcttg

SEQ ID NO: 7668 - RNA, 20 nt, synthetic construct
  source 1..20: mol_type = other RNA
gatcagaataggaggcttgt

SEQ ID NO: 7669 - RNA, 20 nt, synthetic construct
  source 1..20: mol_type = other RNA
atcagaataggaggcttgtg

SEQ ID NO: 7670 - RNA, 20 nt, synthetic construct
  source 1..20: mol_type = other RNA
acaagtggcagctggataaa

SEQ ID NO: 7671 - RNA, 20 nt, synthetic construct
  source 1..20: mol_type = other RNA
atccagctgccacttgttag

SEQ ID NO: 7672 - RNA, 20 nt, synthetic construct
  source 1..20: mol_type = other RNA
atcctctaacaagtggcagc

SEQ ID NO: 7673 - RNA, 20 nt, synthetic construct
  source 1..20: mol_type = other RNA
aaccggcatcctctaacaag

SEQ ID NO: 7674 - RNA, 20 nt, synthetic construct
  source 1..20: mol_type = other RNA
tcagcctgaaagcagaaaac

SEQ ID NO: 7675 - RNA, 20 nt, synthetic construct
  source 1..20: mol_type = other RNA
gtcaccggttttctgctttc

SEQ ID NO: 7676 - RNA, 20 nt, synthetic construct
  source 1..20: mol_type = other RNA
aaagatgttttgtttgtcac

SEQ ID NO: 7677 - RNA, 20 nt, synthetic construct
  source 1..20: mol_type = other RNA
aacaaaacatctttcattac

SEQ ID NO: 7678 - RNA, 20 nt, synthetic construct
  source 1..20: mol_type = other RNA
tcattacaggctcacttaaa

SEQ ID NO: 7679 - RNA, 20 nt, synthetic construct
  source 1..20: mol_type = other RNA
cattacaggctcacttaaaa

SEQ ID NO: 7680 - RNA, 20 nt, synthetic construct
  source 1..20: mol_type = other RNA
attacaggctcacttaaaag

SEQ ID NO: 7681 - RNA, 20 nt, synthetic construct
  source 1..20: mol_type = other RNA
aggctcacttaaaaggggcc

SEQ ID NO: 7682 - RNA, 20 nt, synthetic construct
  source 1..20: mol_type = other RNA
aagtcaagataaaaacagcc

SEQ ID NO: 7683 - RNA, 20 nt, synthetic construct
  source 1..20: mol_type = other RNA
gtatatgagcagaaaacgaa

SEQ ID NO: 7684 - RNA, 20 nt, synthetic construct
  source 1..20: mol_type = other RNA
tatatgagcagaaaacgaat

SEQ ID NO: 7685 - RNA, 20 nt, synthetic construct
  source 1..20: mol_type = other RNA
tgagcagaaaacgaatgggc

SEQ ID NO: 7686 - RNA, 20 nt, synthetic construct
  source 1..20: mol_type = other RNA
ctggcttggggtctgcagga

SEQ ID NO: 7687 - RNA, 20 nt, synthetic construct
  source 1..20: mol_type = other RNA
gcttggggtctgcaggaggg

SEQ ID NO: 7688 - RNA, 20 nt, synthetic construct
  source 1..20: mol_type = other RNA
cctcctgcagaccccaagcc

SEQ ID NO: 7689 - RNA, 20 nt, synthetic construct
  source 1..20: mol_type = other RNA
tgtcactgtcacactgctgc

SEQ ID NO: 7690 - RNA, 20 nt, synthetic construct
  source 1..20: mol_type = other RNA
agtgtgacagtgacaatgcc

SEQ ID NO: 7691 - RNA, 20 nt, synthetic construct
  source 1..20: mol_type = other RNA
tctatgaggatagcaagtcc

SEQ ID NO: 7692 - RNA, 20 nt, synthetic construct
  source 1..20: mol_type = other RNA
ctctatgaggatagcaagtc

SEQ ID NO: 7693 - RNA, 20 nt, synthetic construct
  source 1..20: mol_type = other RNA
tatcctcatagagacagaag

SEQ ID NO: 7694 - RNA, 20 nt, synthetic construct
  source 1..20: mol_type = other RNA
atcctcatagagacagaagt

SEQ ID NO: 7695 - RNA, 20 nt, synthetic construct
  source 1..20: mol_type = other RNA
atagagacagaagtgggcag

SEQ ID NO: 7696 - RNA, 20 nt, synthetic construct
  source 1..20: mol_type = other RNA
tgcccacttctgtctctatg

SEQ ID NO: 7697 - RNA, 20 nt, synthetic construct
  source 1..20: mol_type = other RNA
gacagaagtgggcagaggag

SEQ ID NO: 7698 - RNA, 20 nt, synthetic construct
  source 1..20: mol_type = other RNA
gcagaggagaggcctgagcc

SEQ ID NO: 7699 - RNA, 20 nt, synthetic construct
  source 1..20: mol_type = other RNA
gagccaggcagcgcttacct

SEQ ID NO: 7700 - RNA, 20 nt, synthetic construct
  source 1..20: mol_type = other RNA
agccaggcagcgcttacctc

SEQ ID NO: 7701 - RNA, 20 nt, synthetic construct
  source 1..20: mol_type = other RNA
aggtaagcgctgcctggctc

SEQ ID NO: 7702 - RNA, 20 nt, synthetic construct
  source 1..20: mol_type = other RNA
ggcagcgcttacctcggggc

SEQ ID NO: 7703 - RNA, 20 nt, synthetic construct
  source 1..20: mol_type = other RNA
gccccgaggtaagcgctgcc

SEQ ID NO: 7704 - RNA, 20 nt, synthetic construct
  source 1..20: mol_type = other RNA
ttacctcggggctggagaag

SEQ ID NO: 7705 - RNA, 20 nt, synthetic construct
  source 1..20: mol_type = other RNA
tacctcggggctggagaagt

SEQ ID NO: 7706 - RNA, 20 nt, synthetic construct
  source 1..20: mol_type = other RNA
acctcggggctggagaagtg

SEQ ID NO: 7707 - RNA, 20 nt, synthetic construct
  source 1..20: mol_type = other RNA
cctcggggctggagaagtgg

SEQ ID NO: 7708 - RNA, 20 nt, synthetic construct
  source 1..20: mol_type = other RNA
ctcggggctggagaagtggg

SEQ ID NO: 7709 - RNA, 20 nt, synthetic construct
  source 1..20: mol_type = other RNA
tcggggctggagaagtgggg

SEQ ID NO: 7710 - RNA, 20 nt, synthetic construct
  source 1..20: mol_type = other RNA
cccccacttctccagccccg

SEQ ID NO: 7711 - RNA, 20 nt, synthetic construct
  source 1..20: mol_type = other RNA
cttgctgccctcactctcgc

SEQ ID NO: 7712 - RNA, 20 nt, synthetic construct
  source 1..20: mol_type = other RNA
actctcgctggagctgctct

SEQ ID NO: 7713 - RNA, 20 nt, synthetic construct
  source 1..20: mol_type = other RNA
gagcagctccagcgagagtg

SEQ ID NO: 7714 - RNA, 20 nt, synthetic construct
  source 1..20: mol_type = other RNA
ctcggtctccgagtcagatc

SEQ ID NO: 7715 - RNA, 20 nt, synthetic construct
  source 1..20: mol_type = other RNA
gagcagctccggatctgact

SEQ ID NO: 7716 - RNA, 20 nt, synthetic construct
  source 1..20: mol_type = other RNA
ggagctgctctctgagtcgc

SEQ ID NO: 7717 - RNA, 20 nt, synthetic construct
  source 1..20: mol_type = other RNA
agcgactcagagagcagctc

SEQ ID NO: 7718 - RNA, 20 nt, synthetic construct
  source 1..20: mol_type = other RNA
agcagcagcagcagcagcag

SEQ ID NO: 7719 - RNA, 20 nt, synthetic construct
  source 1..20: mol_type = other RNA
gctgctgctgctgcccttgc

SEQ ID NO: 7720 - RNA, 20 nt, synthetic construct
  source 1..20: mol_type = other RNA
ctgctgctgcccttgctgga

SEQ ID NO: 7721 - RNA, 20 nt, synthetic construct
  source 1..20: mol_type = other RNA
gcccttgctggaaggcaccg

SEQ ID NO: 7722 - RNA, 20 nt, synthetic construct
  source 1..20: mol_type = other RNA
acctcggtgccttccagcaa

SEQ ID NO: 7723 - RNA, 20 nt, synthetic construct
  source 1..20: mol_type = other RNA
aacctcggtgccttccagca

SEQ ID NO: 7724 - RNA, 20 nt, synthetic construct
  source 1..20: mol_type = other RNA
aggcaccgaggttctgcagt

SEQ ID NO: 7725 - RNA, 20 nt, synthetic construct
  source 1..20: mol_type = other RNA
ggcaccgaggttctgcagtt

SEQ ID NO: 7726 - RNA, 20 nt, synthetic construct
  source 1..20: mol_type = other RNA
aggttctgcagttgggctgc

SEQ ID NO: 7727 - RNA, 20 nt, synthetic construct
  source 1..20: mol_type = other RNA
gcagcccaactgcagaacct

SEQ ID NO: 7728 - RNA, 20 nt, synthetic construct
  source 1..20: mol_type = other RNA
gcagttgggctgctggacca

SEQ ID NO: 7729 - RNA, 20 nt, synthetic construct
  source 1..20: mol_type = other RNA
cacggcgctgccagcccgcg

SEQ ID NO: 7730 - RNA, 20 nt, synthetic construct
  source 1..20: mol_type = other RNA
ctcgcgggctggcagcgccg

SEQ ID NO: 7731 - RNA, 20 nt, synthetic construct
  source 1..20: mol_type = other RNA
ctgccagcccgcgaggcccc

SEQ ID NO: 7732 - RNA, 20 nt, synthetic construct
  source 1..20: mol_type = other RNA
tgccagcccgcgaggccccc

SEQ ID NO: 7733 - RNA, 20 nt, synthetic construct
  source 1..20: mol_type = other RNA
ttcccgggggcctcgcgggc

SEQ ID NO: 7734 - RNA, 20 nt, synthetic construct
  source 1..20: mol_type = other RNA
gcgaggcccccgggaagcag

SEQ ID NO: 7735 - RNA, 20 nt, synthetic construct
  source 1..20: mol_type = other RNA
cgaggcccccgggaagcaga

SEQ ID NO: 7736 - RNA, 20 nt, synthetic construct
  source 1..20: mol_type = other RNA
ctgcttcccgggggcctcgc

SEQ ID NO: 7737 - RNA, 20 nt, synthetic construct
  source 1..20: mol_type = other RNA
tctgcttcccgggggcctcg

SEQ ID NO: 7738 - RNA, 20 nt, synthetic construct
  source 1..20: mol_type = other RNA
gcccccgggaagcagaggga

SEQ ID NO: 7739 - RNA, 20 nt, synthetic construct
  source 1..20: mol_type = other RNA
tccttccctctgcttcccgg

SEQ ID NO: 7740 - RNA, 20 nt, synthetic construct
  source 1..20: mol_type = other RNA
ttccttccctctgcttcccg

SEQ ID NO: 7741 - RNA, 20 nt, synthetic construct
  source 1..20: mol_type = other RNA
tttccttccctctgcttccc

SEQ ID NO: 7742 - RNA, 20 nt, synthetic construct
  source 1..20: mol_type = other RNA
ctttccttccctctgcttcc

SEQ ID NO: 7743 - RNA, 20 nt, synthetic construct
  source 1..20: mol_type = other RNA
ggaaagccaagtgagcaaac

SEQ ID NO: 7744 - RNA, 20 nt, synthetic construct
  source 1..20: mol_type = other RNA
tgttttcctgtttgctcact

SEQ ID NO: 7745 - RNA, 20 nt, synthetic construct
  source 1..20: mol_type = other RNA
tagggtgcatgacagcttgg

SEQ ID NO: 7746 - RNA, 20 nt, synthetic construct
  source 1..20: mol_type = other RNA
agctgtcatgcaccctaaag

SEQ ID NO: 7747 - RNA, 20 nt, synthetic construct
  source 1..20: mol_type = other RNA
gctgtcatgcaccctaaaga

SEQ ID NO: 7748 - RNA, 20 nt, synthetic construct
  source 1..20: mol_type = other RNA
ctttagggtgcatgacagct

SEQ ID NO: 7749 - RNA, 20 nt, synthetic construct
  source 1..20: mol_type = other RNA
gtcatgcaccctaaagaggg

SEQ ID NO: 7750 - RNA, 20 nt, synthetic construct
  source 1..20: mol_type = other RNA
atgcaccctaaagagggagg

SEQ ID NO: 7751 - RNA, 20 nt, synthetic construct
  source 1..20: mol_type = other RNA
gcgtgcctcctccctcttta

SEQ ID NO: 7752 - RNA, 20 nt, synthetic construct
  source 1..20: mol_type = other RNA
tgcgtgcctcctccctcttt

SEQ ID NO: 7753 - RNA, 20 nt, synthetic construct
  source 1..20: mol_type = other RNA
tcccagttcagagatacttt

SEQ ID NO: 7754 - RNA, 20 nt, synthetic construct
  source 1..20: mol_type = other RNA
cccagttcagagatacttta

SEQ ID NO: 7755 - RNA, 20 nt, synthetic construct
  source 1..20: mol_type = other RNA
ccctaaagtatctctgaact

SEQ ID NO: 7756 - RNA, 20 nt, synthetic construct
  source 1..20: mol_type = other RNA
tccctaaagtatctctgaac

SEQ ID NO: 7757 - RNA, 20 nt, synthetic construct
  source 1..20: mol_type = other RNA
tgtggcatataattcataat

SEQ ID NO: 7758 - RNA, 20 nt, synthetic construct
  source 1..20: mol_type = other RNA
aattatatgccacaataaat

SEQ ID NO: 7759 - RNA, 20 nt, synthetic construct
  source 1..20: mol_type = other RNA
attatatgccacaataaata

SEQ ID NO: 7760 - RNA, 20 nt, synthetic construct
  source 1..20: mol_type = other RNA
acattgagccctatttattg

SEQ ID NO: 7761 - RNA, 20 nt, synthetic construct
  source 1..20: mol_type = other RNA
tgtacctgtcagagagagcg

SEQ ID NO: 7762 - RNA, 20 nt, synthetic construct
  source 1..20: mol_type = other RNA
ctctccgcgctctctctgac

SEQ ID NO: 7763 - RNA, 20 nt, synthetic construct
  source 1..20: mol_type = other RNA
ccgttctctgagctgcctgc

SEQ ID NO: 7764 - RNA, 20 nt, synthetic construct
  source 1..20: mol_type = other RNA
ccagcaggcagctcagagaa

SEQ ID NO: 7765 - RNA, 20 nt, synthetic construct
  source 1..20: mol_type = other RNA
ctgcctgctggaagaaagaa

SEQ ID NO: 7766 - RNA, 20 nt, synthetic construct
  source 1..20: mol_type = other RNA
tgcctgctggaagaaagaaa

SEQ ID NO: 7767 - RNA, 20 nt, synthetic construct
  source 1..20: mol_type = other RNA
tgccctttctttcttccagc

SEQ ID NO: 7768 - RNA, 20 nt, synthetic construct
  source 1..20: mol_type = other RNA
caaaaatgtgtgtaatgcag

SEQ ID NO: 7769 - RNA, 20 nt, synthetic construct
  source 1..20: mol_type = other RNA
gcaaaaatgtgtgtaatgca

SEQ ID NO: 7770 - RNA, 20 nt, synthetic construct
  source 1..20: mol_type = other RNA
ggcaaaaatgtgtgtaatgc

SEQ ID NO: 7771 - RNA, 20 nt, synthetic construct
  source 1..20: mol_type = other RNA
ttacacacatttttgccatg

SEQ ID NO: 7772 - RNA, 20 nt, synthetic construct
  source 1..20: mol_type = other RNA
attacaaggaagctaagatc

SEQ ID NO: 7773 - RNA, 20 nt, synthetic construct
  source 1..20: mol_type = other RNA
ttccttgtaatacccattgc

SEQ ID NO: 7774 - RNA, 20 nt, synthetic construct
  source 1..20: mol_type = other RNA
gaccagcaatgggtattaca

SEQ ID NO: 7775 - RNA, 20 nt, synthetic construct
  source 1..20: mol_type = other RNA
atgatattgagaccagcaat

SEQ ID NO: 7776 - RNA, 20 nt, synthetic construct
  source 1..20: mol_type = other RNA
tatgatattgagaccagcaa

SEQ ID NO: 7777 - RNA, 20 nt, synthetic construct
  source 1..20: mol_type = other RNA
ataaaaaattacagaattca

SEQ ID NO: 7778 - RNA, 20 nt, synthetic construct
  source 1..20: mol_type = other RNA
attacagaattcaaggctta

SEQ ID NO: 7779 - RNA, 20 nt, synthetic construct
  source 1..20: mol_type = other RNA
ttacagaattcaaggcttaa

SEQ ID NO: 7780 - RNA, 20 nt, synthetic construct
  source 1..20: mol_type = other RNA
tcaaggcttaagggaaatta

SEQ ID NO: 7781 - RNA, 20 nt, synthetic construct
  source 1..20: mol_type = other RNA
caaggcttaagggaaattat

SEQ ID NO: 7782 - RNA, 20 nt, synthetic construct
  source 1..20: mol_type = other RNA
gtgtgagcttctatgcagtt

SEQ ID NO: 7783 - RNA, 20 nt, synthetic construct
  source 1..20: mol_type = other RNA
agtgtgagcttctatgcagt

SEQ ID NO: 7784 - RNA, 20 nt, synthetic construct
  source 1..20: mol_type = other RNA
cagacaaaagaccagcagcc

SEQ ID NO: 7785 - RNA, 20 nt, synthetic construct
  source 1..20: mol_type = other RNA
atggtggcactccaggctgc

SEQ ID NO: 7786 - RNA, 20 nt, synthetic construct
  source 1..20: mol_type = other RNA
tggagtgccaccattcagct

SEQ ID NO: 7787 - RNA, 20 nt, synthetic construct
  source 1..20: mol_type = other RNA
aagctgaatggtggcactcc

SEQ ID NO: 7788 - RNA, 20 nt, synthetic construct
  source 1..20: mol_type = other RNA
cattcagcttggttaacacc

SEQ ID NO: 7789 - RNA, 20 nt, synthetic construct
  source 1..20: mol_type = other RNA
gtgttaaccaagctgaatgg

SEQ ID NO: 7790 - RNA, 20 nt, synthetic construct
  source 1..20: mol_type = other RNA
cgggtgttaaccaagctgaa

SEQ ID NO: 7791 - RNA, 20 nt, synthetic construct
  source 1..20: mol_type = other RNA
aacacccggcacagtccacc

SEQ ID NO: 7792 - RNA, 20 nt, synthetic construct
  source 1..20: mol_type = other RNA
gttacctggtggactgtgcc

SEQ ID NO: 7793 - RNA, 20 nt, synthetic construct
  source 1..20: mol_type = other RNA
agttacctggtggactgtgc

SEQ ID NO: 7794 - RNA, 20 nt, synthetic construct
  source 1..20: mol_type = other RNA
cactggtaacagttacctgg

SEQ ID NO: 7795 - RNA, 20 nt, synthetic construct
  source 1..20: mol_type = other RNA
tgacactggtaacagttacc

SEQ ID NO: 7796 - RNA, 20 nt, synthetic construct
  source 1..20: mol_type = other RNA
gttaccagtgtcacctccaa

SEQ ID NO: 7797 - RNA, 20 nt, synthetic construct
  source 1..20: mol_type = other RNA
tcatcctttggaggtgacac

SEQ ID NO: 7798 - RNA, 20 nt, synthetic construct
  source 1..20: mol_type = other RNA
tttatgtcatcatcctttgg

SEQ ID NO: 7799 - RNA, 20 nt, synthetic construct
  source 1..20: mol_type = other RNA
tcttttatgtcatcatcctt

SEQ ID NO: 7800 - RNA, 20 nt, synthetic construct
  source 1..20: mol_type = other RNA
tgatgaagaggagaatgaac

SEQ ID NO: 7801 - RNA, 20 nt, synthetic construct
  source 1..20: mol_type = other RNA
cttcatcactgcttagctta

SEQ ID NO: 7802 - RNA, 20 nt, synthetic construct
  source 1..20: mol_type = other RNA
taagctaagcagtgatgaag

SEQ ID NO: 7803 - RNA, 20 nt, synthetic construct
  source 1..20: mol_type = other RNA
tcttccagcattctgaaaga

SEQ ID NO: 7804 - RNA, 20 nt, synthetic construct
  source 1..20: mol_type = other RNA
tgttccttctttcagaatgc

SEQ ID NO: 7805 - RNA, 20 nt, synthetic construct
  source 1..20: mol_type = other RNA
ttctgaaagaaggaacaaag

SEQ ID NO: 7806 - RNA, 20 nt, synthetic construct
  source 1..20: mol_type = other RNA
aggaacaaagaggtacaaag

SEQ ID NO: 7807 - RNA, 20 nt, synthetic construct
  source 1..20: mol_type = other RNA
aaagaggtacagatagttag

SEQ ID NO: 7808 - RNA, 20 nt, synthetic construct
  source 1..20: mol_type = other RNA
acaacattaaggtgatattt

SEQ ID NO: 7809 - RNA, 20 nt, synthetic construct
  source 1..20: mol_type = other RNA
ttgctctaataacaacatta

SEQ ID NO: 7810 - RNA, 20 nt, synthetic construct
  source 1..20: mol_type = other RNA
ttgttattagagcaacattt

SEQ ID NO: 7811 - RNA, 20 nt, synthetic construct
  source 1..20: mol_type = other RNA
aagaaggaaagaaaaaaaat

SEQ ID NO: 7812 - RNA, 20 nt, synthetic construct
  source 1..20: mol_type = other RNA
cttcttatgcacttttcctc

SEQ ID NO: 7813 - RNA, 20 nt, synthetic construct
  source 1..20: mol_type = other RNA
cagaggaaaagtgcataaga

SEQ ID NO: 7814 - RNA, 20 nt, synthetic construct
  source 1..20: mol_type = other RNA
acttttcctctggtgcactt

SEQ ID NO: 7815 - RNA, 20 nt, synthetic construct
  source 1..20: mol_type = other RNA
ctatttcctaagtgcaccag

SEQ ID NO: 7816 - RNA, 20 nt, synthetic construct
  source 1..20: mol_type = other RNA
gagggttaatttttatgatg

SEQ ID NO: 7817 - RNA, 20 nt, synthetic construct
  source 1..20: mol_type = other RNA
tgagggttaatttttatgat

SEQ ID NO: 7818 - RNA, 20 nt, synthetic construct
  source 1..20: mol_type = other RNA
gtgagggttaatttttatga

SEQ ID NO: 7819 - RNA, 20 nt, synthetic construct
  source 1..20: mol_type = other RNA
ttagctgatgactgttgtga

SEQ ID NO: 7820 - RNA, 20 nt, synthetic construct
  source 1..20: mol_type = other RNA
caacagtcatcagctaagac

SEQ ID NO: 7821 - RNA, 20 nt, synthetic construct
  source 1..20: mol_type = other RNA
tcagaagatgctgtgttagc

SEQ ID NO: 7822 - RNA, 20 nt, synthetic construct
  source 1..20: mol_type = other RNA
cagaagatgctgtgttagca

SEQ ID NO: 7823 - RNA, 20 nt, synthetic construct
  source 1..20: mol_type = other RNA
tatatttcgaaatagctaga

SEQ ID NO: 7824 - RNA, 20 nt, synthetic construct
  source 1..20: mol_type = other RNA
atatttcgaaatagctagaa

SEQ ID NO: 7825 - RNA, 20 nt, synthetic construct
  source 1..20: mol_type = other RNA
aatagctagaagggaagaat

SEQ ID NO: 7826 - RNA, 20 nt, synthetic construct
  source 1..20: mol_type = other RNA
agaattggaatgttcccaac

SEQ ID NO: 7827 - RNA, 20 nt, synthetic construct
  source 1..20: mol_type = other RNA
atttatcttttcttcctgtt

SEQ ID NO: 7828 - RNA, 20 nt, synthetic construct
  source 1..20: mol_type = other RNA
tatttatcttttcttcctgt

SEQ ID NO: 7829 - RNA, 20 nt, synthetic construct
  source 1..20: mol_type = other RNA
gaagaaaagataaatatttg

SEQ ID NO: 7830 - RNA, 20 nt, synthetic construct
  source 1..20: mol_type = other RNA
atgatcaaatcagggtaact

SEQ ID NO: 7831 - RNA, 20 nt, synthetic construct
  source 1..20: mol_type = other RNA
aatgtgtaatgatcaaatca

SEQ ID NO: 7832 - RNA, 20 nt, synthetic construct
  source 1..20: mol_type = other RNA
caatgtgtaatgatcaaatc

SEQ ID NO: 7833 - RNA, 20 nt, synthetic construct
  source 1..20: mol_type = other RNA
acgtgtgatattttgataca

SEQ ID NO: 7834 - RNA, 20 nt, synthetic construct
  source 1..20: mol_type = other RNA
tacgtgtgatattttgatac

SEQ ID NO: 7835 - RNA, 20 nt, synthetic construct
  source 1..20: mol_type = other RNA
tcttttttattgctattttc

SEQ ID NO: 7836 - RNA, 20 nt, synthetic construct
  source 1..20: mol_type = other RNA
tttttttctctcaaatacat

SEQ ID NO: 7837 - RNA, 20 nt, synthetic construct
  source 1..20: mol_type = other RNA
ttttttctctcaaatacata

SEQ ID NO: 7838 - RNA, 20 nt, synthetic construct
  source 1..20: mol_type = other RNA
tttttctctcaaatacatag

SEQ ID NO: 7839 - RNA, 20 nt, synthetic construct
  source 1..20: mol_type = other RNA
atacataggggcttttcccc

SEQ ID NO: 7840 - RNA, 20 nt, synthetic construct
  source 1..20: mol_type = other RNA
tacataggggcttttcccct

SEQ ID NO: 7841 - RNA, 20 nt, synthetic construct
  source 1..20: mol_type = other RNA
gtggaatgcaaactgcccag

SEQ ID NO: 7842 - RNA, 20 nt, synthetic construct
  source 1..20: mol_type = other RNA
tgtggaatgcaaactgccca

SEQ ID NO: 7843 - RNA, 20 nt, synthetic construct
  source 1..20: mol_type = other RNA
ttgtggaatgcaaactgccc

SEQ ID NO: 7844 - RNA, 20 nt, synthetic construct
  source 1..20: mol_type = other RNA
aaacactaaacaagtaattg

SEQ ID NO: 7845 - RNA, 20 nt, synthetic construct
  source 1..20: mol_type = other RNA
gttttccaagctcccagtgc

SEQ ID NO: 7846 - RNA, 20 nt, synthetic construct
  source 1..20: mol_type = other RNA
ttttccaagctcccagtgct

SEQ ID NO: 7847 - RNA, 20 nt, synthetic construct
  source 1..20: mol_type = other RNA
acagcccagcactgggagct

SEQ ID NO: 7848 - RNA, 20 nt, synthetic construct
  source 1..20: mol_type = other RNA
cggagacacagcccagcact

SEQ ID NO: 7849 - RNA, 20 nt, synthetic construct
  source 1..20: mol_type = other RNA
acggagacacagcccagcac

SEQ ID NO: 7850 - RNA, 20 nt, synthetic construct
  source 1..20: mol_type = other RNA
tgtgtctccgtgcctgcccc

SEQ ID NO: 7851 - RNA, 20 nt, synthetic construct
  source 1..20: mol_type = other RNA
gtgtctccgtgcctgcccca

SEQ ID NO: 7852 - RNA, 20 nt, synthetic construct
  source 1..20: mol_type = other RNA
tgtctccgtgcctgccccag

SEQ ID NO: 7853 - RNA, 20 nt, synthetic construct
  source 1..20: mol_type = other RNA
gcctgccccaggggctttca

SEQ ID NO: 7854 - RNA, 20 nt, synthetic construct
  source 1..20: mol_type = other RNA
gaaagcccctggggcaggca

SEQ ID NO: 7855 - RNA, 20 nt, synthetic construct
  source 1..20: mol_type = other RNA
accatgaaagcccctggggc

SEQ ID NO: 7856 - RNA, 20 nt, synthetic construct
  source 1..20: mol_type = other RNA
ctttaccatgaaagcccctg

SEQ ID NO: 7857 - RNA, 20 nt, synthetic construct
  source 1..20: mol_type = other RNA
tctttaccatgaaagcccct

SEQ ID NO: 7858 - RNA, 20 nt, synthetic construct
  source 1..20: mol_type = other RNA
ctctttaccatgaaagcccc

SEQ ID NO: 7859 - RNA, 20 nt, synthetic construct
  source 1..20: mol_type = other RNA
aactcaagtttatggcttta

SEQ ID NO: 7860 - RNA, 20 nt, synthetic construct
  source 1..20: mol_type = other RNA
tcgctcacaactcaagttta

SEQ ID NO: 7861 - RNA, 20 nt, synthetic construct
  source 1..20: mol_type = other RNA
agttgtgagcgaagcttctt

SEQ ID NO: 7862 - RNA, 20 nt, synthetic construct
  source 1..20: mol_type = other RNA
ccatccatcagtcaaagagc

SEQ ID NO: 7863 - RNA, 20 nt, synthetic construct
  source 1..20: mol_type = other RNA
ccagctctttgactgatgga

SEQ ID NO: 7864 - RNA, 20 nt, synthetic construct
  source 1..20: mol_type = other RNA
ttttccagctctttgactga

SEQ ID NO: 7865 - RNA, 20 nt, synthetic construct
  source 1..20: mol_type = other RNA
gtccccaagatcctacctag

SEQ ID NO: 7866 - RNA, 20 nt, synthetic construct
  source 1..20: mol_type = other RNA
tccccaagatcctacctagt

SEQ ID NO: 7867 - RNA, 20 nt, synthetic construct
  source 1..20: mol_type = other RNA
ccccaagatcctacctagtg

SEQ ID NO: 7868 - RNA, 20 nt, synthetic construct
  source 1..20: mol_type = other RNA
ccccactaggtaggatcttg

SEQ ID NO: 7869 - RNA, 20 nt, synthetic construct
  source 1..20: mol_type = other RNA
tccccactaggtaggatctt

SEQ ID NO: 7870 - RNA, 20 nt, synthetic construct
  source 1..20: mol_type = other RNA
ttccccactaggtaggatct

SEQ ID NO: 7871 - RNA, 20 nt, synthetic construct
  source 1..20: mol_type = other RNA
cctagtggggaaaaccaagc

SEQ ID NO: 7872 - RNA, 20 nt, synthetic construct
  source 1..20: mol_type = other RNA
cttggttttccccactaggt

SEQ ID NO: 7873 - RNA, 20 nt, synthetic construct
  source 1..20: mol_type = other RNA
agtggggaaaaccaagcagg

SEQ ID NO: 7874 - RNA, 20 nt, synthetic construct
  source 1..20: mol_type = other RNA
gtggggaaaaccaagcagga

SEQ ID NO: 7875 - RNA, 20 nt, synthetic construct
  source 1..20: mol_type = other RNA
cctgcttggttttccccact

SEQ ID NO: 7876 - RNA, 20 nt, synthetic construct
  source 1..20: mol_type = other RNA
tcagaaagcgccctcctgct

SEQ ID NO: 7877 - RNA, 20 nt, synthetic construct
  source 1..20: mol_type = other RNA
gctttctgaaaagcctgtga

SEQ ID NO: 7878 - RNA, 20 nt, synthetic construct
  source 1..20: mol_type = other RNA
ggctggggaatcaccttcac

SEQ ID NO: 7879 - RNA, 20 nt, synthetic construct
  source 1..20: mol_type = other RNA
ggtgattccccagcccaccc

SEQ ID NO: 7880 - RNA, 20 nt, synthetic construct
  source 1..20: mol_type = other RNA
ggggggacctgggtgggctg

SEQ ID NO: 7881 - RNA, 20 nt, synthetic construct
  source 1..20: mol_type = other RNA
tggggggacctgggtgggct

SEQ ID NO: 7882 - RNA, 20 nt, synthetic construct
  source 1..20: mol_type = other RNA
atggggggacctgggtgggc

SEQ ID NO: 7883 - RNA, 20 nt, synthetic construct
  source 1..20: mol_type = other RNA
atgaatggggggacctgggt

SEQ ID NO: 7884 - RNA, 20 nt, synthetic construct
  source 1..20: mol_type = other RNA
gatgaatggggggacctggg

SEQ ID NO: 7885 - RNA, 20 nt, synthetic construct
  source 1..20: mol_type = other RNA
aggtccccccattcatcctg

SEQ ID NO: 7886 - RNA, 20 nt, synthetic construct
  source 1..20: mol_type = other RNA
caggatgaatggggggacct

SEQ ID NO: 7887 - RNA, 20 nt, synthetic construct
  source 1..20: mol_type = other RNA
tcaggatgaatggggggacc

SEQ ID NO: 7888 - RNA, 20 nt, synthetic construct
  source 1..20: mol_type = other RNA
gtctcctcaggatgaatggg

SEQ ID NO: 7889 - RNA, 20 nt, synthetic construct
  source 1..20: mol_type = other RNA
tgtctcctcaggatgaatgg

SEQ ID NO: 7890 - RNA, 20 nt, synthetic construct
  source 1..20: mol_type = other RNA
ctgtctcctcaggatgaatg

SEQ ID NO: 7891 - RNA, 20 nt, synthetic construct
  source 1..20: mol_type = other RNA
gctgtctcctcaggatgaat

SEQ ID NO: 7892 - RNA, 20 nt, synthetic construct
  source 1..20: mol_type = other RNA
cgctgtctcctcaggatgaa

SEQ ID NO: 7893 - RNA, 20 nt, synthetic construct
  source 1..20: mol_type = other RNA
tgcttccccgctgtctcctc

SEQ ID NO: 7894 - RNA, 20 nt, synthetic construct
  source 1..20: mol_type = other RNA
acactgtattcttttcagca

SEQ ID NO: 7895 - RNA, 20 nt, synthetic construct
  source 1..20: mol_type = other RNA
ctccacgcagagacgctctg

SEQ ID NO: 7896 - RNA, 20 nt, synthetic construct
  source 1..20: mol_type = other RNA
tccacgcagagacgctctga

SEQ ID NO: 7897 - RNA, 20 nt, synthetic construct
  source 1..20: mol_type = other RNA
cagagacgctctgagggagc

SEQ ID NO: 7898 - RNA, 20 nt, synthetic construct
  source 1..20: mol_type = other RNA
agagacgctctgagggagca

SEQ ID NO: 7899 - RNA, 20 nt, synthetic construct
  source 1..20: mol_type = other RNA
gagacgctctgagggagcag

SEQ ID NO: 7900 - RNA, 20 nt, synthetic construct
  source 1..20: mol_type = other RNA
caggggagagcccacttctg

SEQ ID NO: 7901 - RNA, 20 nt, synthetic construct
  source 1..20: mol_type = other RNA
aggggagagcccacttctga

SEQ ID NO: 7902 - RNA, 20 nt, synthetic construct
  source 1..20: mol_type = other RNA
agcccacttctgagggaccc

SEQ ID NO: 7903 - RNA, 20 nt, synthetic construct
  source 1..20: mol_type = other RNA
gcccacttctgagggaccct

SEQ ID NO: 7904 - RNA, 20 nt, synthetic construct
  source 1..20: mol_type = other RNA
cccacttctgagggaccctg

SEQ ID NO: 7905 - RNA, 20 nt, synthetic construct
  source 1..20: mol_type = other RNA
ccccagggtccctcagaagt

SEQ ID NO: 7906 - RNA, 20 nt, synthetic construct
  source 1..20: mol_type = other RNA
gccccagggtccctcagaag

SEQ ID NO: 7907 - RNA, 20 nt, synthetic construct
  source 1..20: mol_type = other RNA
cactgatgtatggagcccca

SEQ ID NO: 7908 - RNA, 20 nt, synthetic construct
  source 1..20: mol_type = other RNA
acactgatgtatggagcccc

SEQ ID NO: 7909 - RNA, 20 nt, synthetic construct
  source 1..20: mol_type = other RNA
gcgggcttcacactgatgta

SEQ ID NO: 7910 - RNA, 20 nt, synthetic construct
  source 1..20: mol_type = other RNA
cgctgagcccttgtgctcaa

SEQ ID NO: 7911 - RNA, 20 nt, synthetic construct
  source 1..20: mol_type = other RNA
tttgagcacaagggctcagc

SEQ ID NO: 7912 - RNA, 20 nt, synthetic construct
  source 1..20: mol_type = other RNA
ctttgagcacaagggctcag

SEQ ID NO: 7913 - RNA, 20 nt, synthetic construct
  source 1..20: mol_type = other RNA
aatgaggcctttgagcacaa

SEQ ID NO: 7914 - RNA, 20 nt, synthetic construct
  source 1..20: mol_type = other RNA
caatgaggcctttgagcaca

SEQ ID NO: 7915 - RNA, 20 nt, synthetic construct
  source 1..20: mol_type = other RNA
tcattgaagccagcttccaa

SEQ ID NO: 7916 - RNA, 20 nt, synthetic construct
  source 1..20: mol_type = other RNA
tttggaagctggcttcaatg

SEQ ID NO: 7917 - RNA, 20 nt, synthetic construct
  source 1..20: mol_type = other RNA
aggggacagcctttggaagc

SEQ ID NO: 7918 - RNA, 20 nt, synthetic construct
  source 1..20: mol_type = other RNA
acattttaggggacagcctt

SEQ ID NO: 7919 - RNA, 20 nt, synthetic construct
  source 1..20: mol_type = other RNA
ggacactaggtacattttag

SEQ ID NO: 7920 - RNA, 20 nt, synthetic construct
  source 1..20: mol_type = other RNA
aggacactaggtacatttta

SEQ ID NO: 7921 - RNA, 20 nt, synthetic construct
  source 1..20: mol_type = other RNA
aaggacactaggtacatttt

SEQ ID NO: 7922 - RNA, 20 nt, synthetic construct
  source 1..20: mol_type = other RNA
acctagtgtcctttaaaagc

SEQ ID NO: 7923 - RNA, 20 nt, synthetic construct
  source 1..20: mol_type = other RNA
accggcttttaaaggacact

SEQ ID NO: 7924 - RNA, 20 nt, synthetic construct
  source 1..20: mol_type = other RNA
gtcctttaaaagccggttgt

SEQ ID NO: 7925 - RNA, 20 nt, synthetic construct
  source 1..20: mol_type = other RNA
ggcctacaaccggcttttaa

SEQ ID NO: 7926 - RNA, 20 nt, synthetic construct
  source 1..20: mol_type = other RNA
atcagtgataggcctacaac

SEQ ID NO: 7927 - RNA, 20 nt, synthetic construct
  source 1..20: mol_type = other RNA
cagaggcatgtatcagtgat

SEQ ID NO: 7928 - RNA, 20 nt, synthetic construct
  source 1..20: mol_type = other RNA
acatgcctctgaacattcgt

SEQ ID NO: 7929 - RNA, 20 nt, synthetic construct
  source 1..20: mol_type = other RNA
tgactcctacgaatgttcag

SEQ ID NO: 7930 - RNA, 20 nt, synthetic construct
  source 1..20: mol_type = other RNA
ggagtcatttcagtcacttt

SEQ ID NO: 7931 - RNA, 20 nt, synthetic construct
  source 1..20: mol_type = other RNA
gagtcatttcagtcactttt

SEQ ID NO: 7932 - RNA, 20 nt, synthetic construct
  source 1..20: mol_type = other RNA
agtcatttcagtcacttttg

SEQ ID NO: 7933 - RNA, 20 nt, synthetic construct
  source 1..20: mol_type = other RNA
cagtcacttttggggcgaac

SEQ ID NO: 7934 - RNA, 20 nt, synthetic construct
  source 1..20: mol_type = other RNA
agtcacttttggggcgaact

SEQ ID NO: 7935 - RNA, 20 nt, synthetic construct
  source 1..20: mol_type = other RNA
gtcacttttggggcgaactg

SEQ ID NO: 7936 - RNA, 20 nt, synthetic construct
  source 1..20: mol_type = other RNA
tcacttttggggcgaactgg

SEQ ID NO: 7937 - RNA, 20 nt, synthetic construct
  source 1..20: mol_type = other RNA
cacttttggggcgaactggg

SEQ ID NO: 7938 - RNA, 20 nt, synthetic construct
  source 1..20: mol_type = other RNA
cgaactggggggtaaagaac

SEQ ID NO: 7939 - RNA, 20 nt, synthetic construct
  source 1..20: mol_type = other RNA
ctggggggtaaagaactggc

SEQ ID NO: 7940 - RNA, 20 nt, synthetic construct
  source 1..20: mol_type = other RNA
ggtaaagaactggcaggata

SEQ ID NO: 7941 - RNA, 20 nt, synthetic construct
  source 1..20: mol_type = other RNA
agaactggcaggataaggca

SEQ ID NO: 7942 - RNA, 20 nt, synthetic construct
  source 1..20: mol_type = other RNA
ggcaggataaggcatggccc

SEQ ID NO: 7943 - RNA, 20 nt, synthetic construct
  source 1..20: mol_type = other RNA
agacaggtggggcagagcct

SEQ ID NO: 7944 - RNA, 20 nt, synthetic construct
  source 1..20: mol_type = other RNA
tagacaggtggggcagagcc

SEQ ID NO: 7945 - RNA, 20 nt, synthetic construct
  source 1..20: mol_type = other RNA
gccccacctgtctatgcatg

SEQ ID NO: 7946 - RNA, 20 nt, synthetic construct
  source 1..20: mol_type = other RNA
ccccacctgtctatgcatgt

SEQ ID NO: 7947 - RNA, 20 nt, synthetic construct
  source 1..20: mol_type = other RNA
cccacctgtctatgcatgtg

SEQ ID NO: 7948 - RNA, 20 nt, synthetic construct
  source 1..20: mol_type = other RNA
cccacatgcatagacaggtg

SEQ ID NO: 7949 - RNA, 20 nt, synthetic construct
  source 1..20: mol_type = other RNA
ccccacatgcatagacaggt

SEQ ID NO: 7950 - RNA, 20 nt, synthetic construct
  source 1..20: mol_type = other RNA
accccacatgcatagacagg

SEQ ID NO: 7951 - RNA, 20 nt, synthetic construct
  source 1..20: mol_type = other RNA
ctcaccccacatgcatagac

SEQ ID NO: 7952 - RNA, 20 nt, synthetic construct
  source 1..20: mol_type = other RNA
caaatagggaaatggggtca

SEQ ID NO: 7953 - RNA, 20 nt, synthetic construct
  source 1..20: mol_type = other RNA
acaaatagggaaatggggtc

SEQ ID NO: 7954 - RNA, 20 nt, synthetic construct
  source 1..20: mol_type = other RNA
actgcacaaatagggaaatg

SEQ ID NO: 7955 - RNA, 20 nt, synthetic construct
  source 1..20: mol_type = other RNA
cactgcacaaatagggaaat

SEQ ID NO: 7956 - RNA, 20 nt, synthetic construct
  source 1..20: mol_type = other RNA
tcactgcacaaatagggaaa

SEQ ID NO: 7957 - RNA, 20 nt, synthetic construct
  source 1..20: mol_type = other RNA
aacacgtcactgcacaaata

SEQ ID NO: 7958 - RNA, 20 nt, synthetic construct
  source 1..20: mol_type = other RNA
taacacgtcactgcacaaat

SEQ ID NO: 7959 - RNA, 20 nt, synthetic construct
  source 1..20: mol_type = other RNA
tgtgcagtgacgtgttatag

SEQ ID NO: 7960 - RNA, 20 nt, synthetic construct
  source 1..20: mol_type = other RNA
gtgcagtgacgtgttataga

SEQ ID NO: 7961 - RNA, 20 nt, synthetic construct
  source 1..20: mol_type = other RNA
tgttatagagggcaatccta

SEQ ID NO: 7962 - RNA, 20 nt, synthetic construct
  source 1..20: mol_type = other RNA
ctaaagcaggattcaacctt

SEQ ID NO: 7963 - RNA, 20 nt, synthetic construct
  source 1..20: mol_type = other RNA
ctcacaacggaatctaaagc

SEQ ID NO: 7964 - RNA, 20 nt, synthetic construct
  source 1..20: mol_type = other RNA
actctccccccatcttccat

SEQ ID NO: 7965 - RNA, 20 nt, synthetic construct
  source 1..20: mol_type = other RNA
ttattccaatggaagatggg

SEQ ID NO: 7966 - RNA, 20 nt, synthetic construct
  source 1..20: mol_type = other RNA
cttattccaatggaagatgg

SEQ ID NO: 7967 - RNA, 20 nt, synthetic construct
  source 1..20: mol_type = other RNA
tcttattccaatggaagatg

SEQ ID NO: 7968 - RNA, 20 nt, synthetic construct
  source 1..20: mol_type = other RNA
ttcttattccaatggaagat

SEQ ID NO: 7969 - RNA, 20 nt, synthetic construct
  source 1..20: mol_type = other RNA
attcttattccaatggaaga

SEQ ID NO: 7970 - RNA, 20 nt, synthetic construct
  source 1..20: mol_type = other RNA
attggaataagaatgcttga

SEQ ID NO: 7971 - RNA, 20 nt, synthetic construct
  source 1..20: mol_type = other RNA
ttggaataagaatgcttgaa

SEQ ID NO: 7972 - RNA, 20 nt, synthetic construct
  source 1..20: mol_type = other RNA
ttcaagcattcttattccaa

SEQ ID NO: 7973 - RNA, 20 nt, synthetic construct
  source 1..20: mol_type = other RNA
aataagaatgcttgaaggga

SEQ ID NO: 7974 - RNA, 20 nt, synthetic construct
  source 1..20: mol_type = other RNA
ataagaatgcttgaagggaa

SEQ ID NO: 7975 - RNA, 20 nt, synthetic construct
  source 1..20: mol_type = other RNA
taagaatgcttgaagggaag

SEQ ID NO: 7976 - RNA, 20 nt, synthetic construct
  source 1..20: mol_type = other RNA
ggtgtgtttcctcaacgcct

SEQ ID NO: 7977 - RNA, 20 nt, synthetic construct
  source 1..20: mol_type = other RNA
tttcctcaacgcctaggata

SEQ ID NO: 7978 - RNA, 20 nt, synthetic construct
  source 1..20: mol_type = other RNA
atgccttatcctaggcgttg

SEQ ID NO: 7979 - RNA, 20 nt, synthetic construct
  source 1..20: mol_type = other RNA
atgggcttatgccttatcct

SEQ ID NO: 7980 - RNA, 20 nt, synthetic construct
  source 1..20: mol_type = other RNA
gcataagcccatcattacta

SEQ ID NO: 7981 - RNA, 20 nt, synthetic construct
  source 1..20: mol_type = other RNA
ggtaattccttagtaatgat

SEQ ID NO: 7982 - RNA, 20 nt, synthetic construct
  source 1..20: mol_type = other RNA
tggtaattccttagtaatga

SEQ ID NO: 7983 - RNA, 20 nt, synthetic construct
  source 1..20: mol_type = other RNA
aagaattctaaaatgcctcg

SEQ ID NO: 7984 - RNA, 20 nt, synthetic construct
  source 1..20: mol_type = other RNA
agttgttttgagaaaccaca

SEQ ID NO: 7985 - RNA, 20 nt, synthetic construct
  source 1..20: mol_type = other RNA
gagaaaccacaaggcagcgc

SEQ ID NO: 7986 - RNA, 20 nt, synthetic construct
  source 1..20: mol_type = other RNA
agaaaccacaaggcagcgct

SEQ ID NO: 7987 - RNA, 20 nt, synthetic construct
  source 1..20: mol_type = other RNA
gaaaccacaaggcagcgctg

SEQ ID NO: 7988 - RNA, 20 nt, synthetic construct
  source 1..20: mol_type = other RNA
gattccccagcgctgccttg

SEQ ID NO: 7989 - RNA, 20 nt, synthetic construct
  source 1..20: mol_type = other RNA
tccagcttgttcttcagcct

SEQ ID NO: 7990 - RNA, 20 nt, synthetic construct
  source 1..20: mol_type = other RNA
ccagcttgttcttcagcctt

SEQ ID NO: 7991 - RNA, 20 nt, synthetic construct
  source 1..20: mol_type = other RNA
cagcttgttcttcagccttg

SEQ ID NO: 7992 - RNA, 20 nt, synthetic construct
  source 1..20: mol_type = other RNA
cttgttcttcagccttgggg

SEQ ID NO: 7993 - RNA, 20 nt, synthetic construct
  source 1..20: mol_type = other RNA
cccaaggctgaagaacaagc

SEQ ID NO: 7994 - RNA, 20 nt, synthetic construct
  source 1..20: mol_type = other RNA
aattttctgtttcctcccca

SEQ ID NO: 7995 - RNA, 20 nt, synthetic construct
  source 1..20: mol_type = other RNA
gccacacctttcaagctccc

SEQ ID NO: 7996 - RNA, 20 nt, synthetic construct
  source 1..20: mol_type = other RNA
tccagggagcttgaaaggtg

SEQ ID NO: 7997 - RNA, 20 nt, synthetic construct
  source 1..20: mol_type = other RNA
acttctccagggagcttgaa

SEQ ID NO: 7998 - RNA, 20 nt, synthetic construct
  source 1..20: mol_type = other RNA
aaagtgtggggacttctcca

SEQ ID NO: 7999 - RNA, 20 nt, synthetic construct
  source 1..20: mol_type = other RNA
gaaagtgtggggacttctcc

SEQ ID NO: 8000 - RNA, 20 nt, synthetic construct
  source 1..20: mol_type = other RNA
cactttcgtcaagactgcat

SEQ ID NO: 8001 - RNA, 20 nt, synthetic construct
  source 1..20: mol_type = other RNA
tgcagtcttgacgaaagtgt

SEQ ID NO: 8002 - RNA, 20 nt, synthetic construct
  source 1..20: mol_type = other RNA
atgcagtcttgacgaaagtg

SEQ ID NO: 8003 - RNA, 20 nt, synthetic construct
  source 1..20: mol_type = other RNA
gactgcataggatagtgtgc

SEQ ID NO: 8004 - RNA, 20 nt, synthetic construct
  source 1..20: mol_type = other RNA
actgcataggatagtgtgct

SEQ ID NO: 8005 - RNA, 20 nt, synthetic construct
  source 1..20: mol_type = other RNA
gtgctgggttttctgtctag

SEQ ID NO: 8006 - RNA, 20 nt, synthetic construct
  source 1..20: mol_type = other RNA
ttttctgtctagtggcaact

SEQ ID NO: 8007 - RNA, 20 nt, synthetic construct
  source 1..20: mol_type = other RNA
tagaaaggagtgcttcaaag

SEQ ID NO: 8008 - RNA, 20 nt, synthetic construct
  source 1..20: mol_type = other RNA
atagaaaggagtgcttcaaa

SEQ ID NO: 8009 - RNA, 20 nt, synthetic construct
  source 1..20: mol_type = other RNA
gaagcactcctttctatcac

SEQ ID NO: 8010 - RNA, 20 nt, synthetic construct
  source 1..20: mol_type = other RNA
aagcactcctttctatcaca

SEQ ID NO: 8011 - RNA, 20 nt, synthetic construct
  source 1..20: mol_type = other RNA
agcactcctttctatcacag

SEQ ID NO: 8012 - RNA, 20 nt, synthetic construct
  source 1..20: mol_type = other RNA
ctcctttctatcacaggggc

SEQ ID NO: 8013 - RNA, 20 nt, synthetic construct
  source 1..20: mol_type = other RNA
ctttctatcacaggggctgg

SEQ ID NO: 8014 - RNA, 20 nt, synthetic construct
  source 1..20: mol_type = other RNA
ctccagcccctgtgatagaa

SEQ ID NO: 8015 - RNA, 20 nt, synthetic construct
  source 1..20: mol_type = other RNA
tatcacaggggctggaggcc

SEQ ID NO: 8016 - RNA, 20 nt, synthetic construct
  source 1..20: mol_type = other RNA
atcacaggggctggaggcct

SEQ ID NO: 8017 - RNA, 20 nt, synthetic construct
  source 1..20: mol_type = other RNA
tctggggaaatgtagttccc

SEQ ID NO: 8018 - RNA, 20 nt, synthetic construct
  source 1..20: mol_type = other RNA
tccccagaatccctgccgat

SEQ ID NO: 8019 - RNA, 20 nt, synthetic construct
  source 1..20: mol_type = other RNA
ccccagaatccctgccgata

SEQ ID NO: 8020 - RNA, 20 nt, synthetic construct
  source 1..20: mol_type = other RNA
ccctatcggcagggattctg

SEQ ID NO: 8021 - RNA, 20 nt, synthetic construct
  source 1..20: mol_type = other RNA
accctatcggcagggattct

SEQ ID NO: 8022 - RNA, 20 nt, synthetic construct
  source 1..20: mol_type = other RNA
atccctgccgatagggtttt

SEQ ID NO: 8023 - RNA, 20 nt, synthetic construct
  source 1..20: mol_type = other RNA
aaccaaaaaccctatcggca

SEQ ID NO: 8024 - RNA, 20 nt, synthetic construct
  source 1..20: mol_type = other RNA
taaccaaaaaccctatcggc

SEQ ID NO: 8025 - RNA, 20 nt, synthetic construct
  source 1..20: mol_type = other RNA
catttaaccaaaaaccctat

SEQ ID NO: 8026 - RNA, 20 nt, synthetic construct
  source 1..20: mol_type = other RNA
ggttaaatgttgccagtgag

SEQ ID NO: 8027 - RNA, 20 nt, synthetic construct
  source 1..20: mol_type = other RNA
ccagtgagaggcacctgaat

SEQ ID NO: 8028 - RNA, 20 nt, synthetic construct
  source 1..20: mol_type = other RNA
cagtgagaggcacctgaata

SEQ ID NO: 8029 - RNA, 20 nt, synthetic construct
  source 1..20: mol_type = other RNA
cctattcaggtgcctctcac

SEQ ID NO: 8030 - RNA, 20 nt, synthetic construct
  source 1..20: mol_type = other RNA
agaggcacctgaatagggct

SEQ ID NO: 8031 - RNA, 20 nt, synthetic construct
  source 1..20: mol_type = other RNA
tgattttccaagccctattc

SEQ ID NO: 8032 - RNA, 20 nt, synthetic construct
  source 1..20: mol_type = other RNA
cagaagcctttactactccc

SEQ ID NO: 8033 - RNA, 20 nt, synthetic construct
  source 1..20: mol_type = other RNA
cactgtcctgggagtagtaa

SEQ ID NO: 8034 - RNA, 20 nt, synthetic construct
  source 1..20: mol_type = other RNA
tactcccaggacagtgaagc

SEQ ID NO: 8035 - RNA, 20 nt, synthetic construct
  source 1..20: mol_type = other RNA
tgcacctgcttcactgtcct

SEQ ID NO: 8036 - RNA, 20 nt, synthetic construct
  source 1..20: mol_type = other RNA
ctgcacctgcttcactgtcc

SEQ ID NO: 8037 - RNA, 20 nt, synthetic construct
  source 1..20: mol_type = other RNA
ggtgcagaagcttcagcaga

SEQ ID NO: 8038 - RNA, 20 nt, synthetic construct
  source 1..20: mol_type = other RNA
ttcagcagatggcagatacg

SEQ ID NO: 8039 - RNA, 20 nt, synthetic construct
  source 1..20: mol_type = other RNA
cagatacgaggttctgtgag

SEQ ID NO: 8040 - RNA, 20 nt, synthetic construct
  source 1..20: mol_type = other RNA
aggttctgtgagtggcttcc

SEQ ID NO: 8041 - RNA, 20 nt, synthetic construct
  source 1..20: mol_type = other RNA
attattcacagaagggtgcc

SEQ ID NO: 8042 - RNA, 20 nt, synthetic construct
  source 1..20: mol_type = other RNA
cttctgtgaataatgcctgc

SEQ ID NO: 8043 - RNA, 20 nt, synthetic construct
  source 1..20: mol_type = other RNA
agcaggcattattcacagaa

SEQ ID NO: 8044 - RNA, 20 nt, synthetic construct
  source 1..20: mol_type = other RNA
cagcaggcattattcacaga

SEQ ID NO: 8045 - RNA, 20 nt, synthetic construct
  source 1..20: mol_type = other RNA
taatctcagatgtctccagc

SEQ ID NO: 8046 - RNA, 20 nt, synthetic construct
  source 1..20: mol_type = other RNA
gaaatgactttctgaactga

SEQ ID NO: 8047 - RNA, 20 nt, synthetic construct
  source 1..20: mol_type = other RNA
actgatggctgatttcctgt

SEQ ID NO: 8048 - RNA, 20 nt, synthetic construct
  source 1..20: mol_type = other RNA
tcctgttggtcccccttccc

SEQ ID NO: 8049 - RNA, 20 nt, synthetic construct
  source 1..20: mol_type = other RNA
gccagggaagggggaccaac

SEQ ID NO: 8050 - RNA, 20 nt, synthetic construct
  source 1..20: mol_type = other RNA
cccttccctggccctcctga

SEQ ID NO: 8051 - RNA, 20 nt, synthetic construct
  source 1..20: mol_type = other RNA
ccttccctggccctcctgat

SEQ ID NO: 8052 - RNA, 20 nt, synthetic construct
  source 1..20: mol_type = other RNA
atcaggagggccagggaagg

SEQ ID NO: 8053 - RNA, 20 nt, synthetic construct
  source 1..20: mol_type = other RNA
catcaggagggccagggaag

SEQ ID NO: 8054 - RNA, 20 nt, synthetic construct
  source 1..20: mol_type = other RNA
ccatcaggagggccagggaa

SEQ ID NO: 8055 - RNA, 20 nt, synthetic construct
  source 1..20: mol_type = other RNA
cctggccctcctgatgggtt

SEQ ID NO: 8056 - RNA, 20 nt, synthetic construct
  source 1..20: mol_type = other RNA
gccctcctgatgggtttgga

SEQ ID NO: 8057 - RNA, 20 nt, synthetic construct
  source 1..20: mol_type = other RNA
ccaaacccatcaggagggcc

SEQ ID NO: 8058 - RNA, 20 nt, synthetic construct
  source 1..20: mol_type = other RNA
gccttccaaacccatcagga

SEQ ID NO: 8059 - RNA, 20 nt, synthetic construct
  source 1..20: mol_type = other RNA
tgccttccaaacccatcagg

SEQ ID NO: 8060 - RNA, 20 nt, synthetic construct
  source 1..20: mol_type = other RNA
tagtgccttccaaacccatc

SEQ ID NO: 8061 - RNA, 20 nt, synthetic construct
  source 1..20: mol_type = other RNA
tcaagtagacacttaacata

SEQ ID NO: 8062 - RNA, 20 nt, synthetic construct
  source 1..20: mol_type = other RNA
ttcaagtagacacttaacat

SEQ ID NO: 8063 - RNA, 20 nt, synthetic construct
  source 1..20: mol_type = other RNA
tctacttgaaatacctagag

SEQ ID NO: 8064 - RNA, 20 nt, synthetic construct
  source 1..20: mol_type = other RNA
tggagaagagaaaccactct

SEQ ID NO: 8065 - RNA, 20 nt, synthetic construct
  source 1..20: mol_type = other RNA
acacatcagtcagtttgatc

SEQ ID NO: 8066 - RNA, 20 nt, synthetic construct
  source 1..20: mol_type = other RNA
agctctgcagtcagaaagcc

SEQ ID NO: 8067 - RNA, 20 nt, synthetic construct
  source 1..20: mol_type = other RNA
tggatagaaatcaataaacc

SEQ ID NO: 8068 - RNA, 20 nt, synthetic construct
  source 1..20: mol_type = other RNA
ctagcatgaggtacagcatc

SEQ ID NO: 8069 - RNA, 20 nt, synthetic construct
  source 1..20: mol_type = other RNA
ataaggacacaactagcatg

SEQ ID NO: 8070 - RNA, 20 nt, synthetic construct
  source 1..20: mol_type = other RNA
aactttaagttctttgcata

SEQ ID NO: 8071 - RNA, 20 nt, synthetic construct
  source 1..20: mol_type = other RNA
ctgtttcctcatctgtaaaa

SEQ ID NO: 8072 - RNA, 20 nt, synthetic construct
  source 1..20: mol_type = other RNA
tttacagatgaggaaacaga

SEQ ID NO: 8073 - RNA, 20 nt, synthetic construct
  source 1..20: mol_type = other RNA
gtttttccattttacagatg

SEQ ID NO: 8074 - RNA, 20 nt, synthetic construct
  source 1..20: mol_type = other RNA
aacgagagtgtttacctcct

SEQ ID NO: 8075 - RNA, 20 nt, synthetic construct
  source 1..20: mol_type = other RNA
ttttctacaacattcctagg

SEQ ID NO: 8076 - RNA, 20 nt, synthetic construct
  source 1..20: mol_type = other RNA
acattttctacaacattcct

SEQ ID NO: 8077 - RNA, 20 nt, synthetic construct
  source 1..20: mol_type = other RNA
aaaacattttatacagtgtc

SEQ ID NO: 8078 - RNA, 20 nt, synthetic construct
  source 1..20: mol_type = other RNA
taaatattcagtattctaac

SEQ ID NO: 8079 - RNA, 20 nt, synthetic construct
  source 1..20: mol_type = other RNA
ttgttgtcacgagatggaat

SEQ ID NO: 8080 - RNA, 20 nt, synthetic construct
  source 1..20: mol_type = other RNA
gttgttgtcacgagatggaa

SEQ ID NO: 8081 - RNA, 20 nt, synthetic construct
  source 1..20: mol_type = other RNA
acatagttgttgtcacgaga

SEQ ID NO: 8082 - RNA, 20 nt, synthetic construct
  source 1..20: mol_type = other RNA
aagaaaaagaaaaggaaaaa

SEQ ID NO: 8083 - RNA, 20 nt, synthetic construct
  source 1..20: mol_type = other RNA
aaaaaagaaagaaaaagaaa

SEQ ID NO: 8084 - RNA, 20 nt, synthetic construct
  source 1..20: mol_type = other RNA
tctcactttgttgcccacgc

SEQ ID NO: 8085 - RNA, 20 nt, synthetic construct
  source 1..20: mol_type = other RNA
ttgcccacgctggagtgcag

SEQ ID NO: 8086 - RNA, 20 nt, synthetic construct
  source 1..20: mol_type = other RNA
acaccactgcactccagcgt

SEQ ID NO: 8087 - RNA, 20 nt, synthetic construct
  source 1..20: mol_type = other RNA
cacaccactgcactccagcg

SEQ ID NO: 8088 - RNA, 20 nt, synthetic construct
  source 1..20: mol_type = other RNA
cactgcagccttgacctccc

SEQ ID NO: 8089 - RNA, 20 nt, synthetic construct
  source 1..20: mol_type = other RNA
cacttgagcctgggaggtca

SEQ ID NO: 8090 - RNA, 20 nt, synthetic construct
  source 1..20: mol_type = other RNA
gaggatcacttgagcctggg

SEQ ID NO: 8091 - RNA, 20 nt, synthetic construct
  source 1..20: mol_type = other RNA
caggaggatcacttgagcct

SEQ ID NO: 8092 - RNA, 20 nt, synthetic construct
  source 1..20: mol_type = other RNA
gcaggaggatcacttgagcc

SEQ ID NO: 8093 - RNA, 20 nt, synthetic construct
  source 1..20: mol_type = other RNA
acttggggggctgaggcagg

SEQ ID NO: 8094 - RNA, 20 nt, synthetic construct
  source 1..20: mol_type = other RNA
gcctcagccccccaagtagc

SEQ ID NO: 8095 - RNA, 20 nt, synthetic construct
  source 1..20: mol_type = other RNA
gctacttggggggctgaggc

SEQ ID NO: 8096 - RNA, 20 nt, synthetic construct
  source 1..20: mol_type = other RNA
tccagctacttggggggctg

SEQ ID NO: 8097 - RNA, 20 nt, synthetic construct
  source 1..20: mol_type = other RNA
ccccaagtagctggaactat

SEQ ID NO: 8098 - RNA, 20 nt, synthetic construct
  source 1..20: mol_type = other RNA
caagtagctggaactatagg

SEQ ID NO: 8099 - RNA, 20 nt, synthetic construct
  source 1..20: mol_type = other RNA
ctatagttccagctacttgg

SEQ ID NO: 8100 - RNA, 20 nt, synthetic construct
  source 1..20: mol_type = other RNA
cctatagttccagctacttg

SEQ ID NO: 8101 - RNA, 20 nt, synthetic construct
  source 1..20: mol_type = other RNA
acctatagttccagctactt

SEQ ID NO: 8102 - RNA, 20 nt, synthetic construct
  source 1..20: mol_type = other RNA
cacctatagttccagctact

SEQ ID NO: 8103 - RNA, 20 nt, synthetic construct
  source 1..20: mol_type = other RNA
tataggtggcccaccatgcc

SEQ ID NO: 8104 - RNA, 20 nt, synthetic construct
  source 1..20: mol_type = other RNA
catgcctggctaatttttgt

SEQ ID NO: 8105 - RNA, 20 nt, synthetic construct
  source 1..20: mol_type = other RNA
caaaaattagccaggcatgg

SEQ ID NO: 8106 - RNA, 20 nt, synthetic construct
  source 1..20: mol_type = other RNA
ctacaaaaattagccaggca

SEQ ID NO: 8107 - RNA, 20 nt, synthetic construct
  source 1..20: mol_type = other RNA
cgtccctacaaaaattagcc

SEQ ID NO: 8108 - RNA, 20 nt, synthetic construct
  source 1..20: mol_type = other RNA
gaggttttgttatgttgccc

SEQ ID NO: 8109 - RNA, 20 nt, synthetic construct
  source 1..20: mol_type = other RNA
ttttgttatgttgcccaggc

SEQ ID NO: 8110 - RNA, 20 nt, synthetic construct
  source 1..20: mol_type = other RNA
ccaggctggtctcaaacccc

SEQ ID NO: 8111 - RNA, 20 nt, synthetic construct
  source 1..20: mol_type = other RNA
caggctggtctcaaacccct

SEQ ID NO: 8112 - RNA, 20 nt, synthetic construct
  source 1..20: mol_type = other RNA
caggggtttgagaccagcct

SEQ ID NO: 8113 - RNA, 20 nt, synthetic construct
  source 1..20: mol_type = other RNA
ccaggggtttgagaccagcc

SEQ ID NO: 8114 - RNA, 20 nt, synthetic construct
  source 1..20: mol_type = other RNA
ggtggatcacttgagcccag

SEQ ID NO: 8115 - RNA, 20 nt, synthetic construct
  source 1..20: mol_type = other RNA
aggtggatcacttgagccca

SEQ ID NO: 8116 - RNA, 20 nt, synthetic construct
  source 1..20: mol_type = other RNA
caggtggatcacttgagccc

SEQ ID NO: 8117 - RNA, 20 nt, synthetic construct
  source 1..20: mol_type = other RNA
ctttgggaggctgaggcagg

SEQ ID NO: 8118 - RNA, 20 nt, synthetic construct
  source 1..20: mol_type = other RNA
gcctcagcctcccaaagtgc

SEQ ID NO: 8119 - RNA, 20 nt, synthetic construct
  source 1..20: mol_type = other RNA
cctcagcctcccaaagtgct

SEQ ID NO: 8120 - RNA, 20 nt, synthetic construct
  source 1..20: mol_type = other RNA
gcactttgggaggctgaggc

SEQ ID NO: 8121 - RNA, 20 nt, synthetic construct
  source 1..20: mol_type = other RNA
cccagcactttgggaggctg

SEQ ID NO: 8122 - RNA, 20 nt, synthetic construct
  source 1..20: mol_type = other RNA
tataatcccagcactttggg

SEQ ID NO: 8123 - RNA, 20 nt, synthetic construct
  source 1..20: mol_type = other RNA
ggctataatcccagcacttt

SEQ ID NO: 8124 - RNA, 20 nt, synthetic construct
  source 1..20: mol_type = other RNA
tggctataatcccagcactt

SEQ ID NO: 8125 - RNA, 20 nt, synthetic construct
  source 1..20: mol_type = other RNA
tctctgttagagaaagtaaa

SEQ ID NO: 8126 - RNA, 20 nt, synthetic construct
  source 1..20: mol_type = other RNA
acctccgacgagcacattct

SEQ ID NO: 8127 - RNA, 20 nt, synthetic construct
  source 1..20: mol_type = other RNA
tagaatgtgctcgtcggagg

SEQ ID NO: 8128 - RNA, 20 nt, synthetic construct
  source 1..20: mol_type = other RNA
acctagaatgtgctcgtcgg

SEQ ID NO: 8129 - RNA, 20 nt, synthetic construct
  source 1..20: mol_type = other RNA
ggcacctagaatgtgctcgt

SEQ ID NO: 8130 - RNA, 20 nt, synthetic construct
  source 1..20: mol_type = other RNA
cttcttcagttttatatctc

SEQ ID NO: 8131 - RNA, 20 nt, synthetic construct
  source 1..20: mol_type = other RNA
tcaagtgtctcactgcttat

SEQ ID NO: 8132 - RNA, 20 nt, synthetic construct
  source 1..20: mol_type = other RNA
caagtgtctcactgcttatt

SEQ ID NO: 8133 - RNA, 20 nt, synthetic construct
  source 1..20: mol_type = other RNA
agcagaaaagaaagccagcg

SEQ ID NO: 8134 - RNA, 20 nt, synthetic construct
  source 1..20: mol_type = other RNA
cagcgaggtgataaatacta

SEQ ID NO: 8135 - RNA, 20 nt, synthetic construct
  source 1..20: mol_type = other RNA
agcgaggtgataaatactat

SEQ ID NO: 8136 - RNA, 20 nt, synthetic construct
  source 1..20: mol_type = other RNA
catagtatttatcacctcgc

SEQ ID NO: 8137 - RNA, 20 nt, synthetic construct
  source 1..20: mol_type = other RNA
tgtctgacaaggaaaaaaga

SEQ ID NO: 8138 - RNA, 20 nt, synthetic construct
  source 1..20: mol_type = other RNA
ttttccttgtcagacaatcc

SEQ ID NO: 8139 - RNA, 20 nt, synthetic construct
  source 1..20: mol_type = other RNA
agggccgggattgtctgaca

SEQ ID NO: 8140 - RNA, 20 nt, synthetic construct
  source 1..20: mol_type = other RNA
caaggaaaaataaaagggcc

SEQ ID NO: 8141 - RNA, 20 nt, synthetic construct
  source 1..20: mol_type = other RNA
acaaggaaaaataaaagggc

SEQ ID NO: 8142 - RNA, 20 nt, synthetic construct
  source 1..20: mol_type = other RNA
aactacaaggaaaaataaaa

SEQ ID NO: 8143 - RNA, 20 nt, synthetic construct
  source 1..20: mol_type = other RNA
aaactacaaggaaaaataaa

SEQ ID NO: 8144 - RNA, 20 nt, synthetic construct
  source 1..20: mol_type = other RNA
gactgaagaataaaactaca

SEQ ID NO: 8145 - RNA, 20 nt, synthetic construct
  source 1..20: mol_type = other RNA
aaggacactggggaacttgt

SEQ ID NO: 8146 - RNA, 20 nt, synthetic construct
  source 1..20: mol_type = other RNA
ataaatttggaaggacactg

SEQ ID NO: 8147 - RNA, 20 nt, synthetic construct
  source 1..20: mol_type = other RNA
tataaatttggaaggacact

SEQ ID NO: 8148 - RNA, 20 nt, synthetic construct
  source 1..20: mol_type = other RNA
ctataaatttggaaggacac

SEQ ID NO: 8149 - RNA, 20 nt, synthetic construct
  source 1..20: mol_type = other RNA
tccaaatttatagtcacgtg

SEQ ID NO: 8150 - RNA, 20 nt, synthetic construct
  source 1..20: mol_type = other RNA
ccaaatttatagtcacgtgt

SEQ ID NO: 8151 - RNA, 20 nt, synthetic construct
  source 1..20: mol_type = other RNA
cacgtgactataaatttgga

SEQ ID NO: 8152 - RNA, 20 nt, synthetic construct
  source 1..20: mol_type = other RNA
cccacacgtgactataaatt

SEQ ID NO: 8153 - RNA, 20 nt, synthetic construct
  source 1..20: mol_type = other RNA
tgggacacagtccactctac

SEQ ID NO: 8154 - RNA, 20 nt, synthetic construct
  source 1..20: mol_type = other RNA
gtccactctacaggctctat

SEQ ID NO: 8155 - RNA, 20 nt, synthetic construct
  source 1..20: mol_type = other RNA
ctctacaggctctatcggca

SEQ ID NO: 8156 - RNA, 20 nt, synthetic construct
  source 1..20: mol_type = other RNA
tgccgatagagcctgtagag

SEQ ID NO: 8157 - RNA, 20 nt, synthetic construct
  source 1..20: mol_type = other RNA
gctctatcggcatggactgt

SEQ ID NO: 8158 - RNA, 20 nt, synthetic construct
  source 1..20: mol_type = other RNA
ctctatcggcatggactgta

SEQ ID NO: 8159 - RNA, 20 nt, synthetic construct
  source 1..20: mol_type = other RNA
tctatcggcatggactgtag

SEQ ID NO: 8160 - RNA, 20 nt, synthetic construct
  source 1..20: mol_type = other RNA
ctatcggcatggactgtagg

SEQ ID NO: 8161 - RNA, 20 nt, synthetic construct
  source 1..20: mol_type = other RNA
gagaatgacccgctttatgt

SEQ ID NO: 8162 - RNA, 20 nt, synthetic construct
  source 1..20: mol_type = other RNA
gttgacttccaacataaagc

SEQ ID NO: 8163 - RNA, 20 nt, synthetic construct
  source 1..20: mol_type = other RNA
tgttgacttccaacataaag

SEQ ID NO: 8164 - RNA, 20 nt, synthetic construct
  source 1..20: mol_type = other RNA
gtcaacagctctgagaatta

SEQ ID NO: 8165 - RNA, 20 nt, synthetic construct
  source 1..20: mol_type = other RNA
agctttaagttatgagtctt

SEQ ID NO: 8166 - RNA, 20 nt, synthetic construct
  source 1..20: mol_type = other RNA
agagactaaatgagcttagg

SEQ ID NO: 8167 - RNA, 20 nt, synthetic construct
  source 1..20: mol_type = other RNA
aggagagactaaatgagctt

SEQ ID NO: 8168 - RNA, 20 nt, synthetic construct
  source 1..20: mol_type = other RNA
ctccttccccaaatgtcttg

SEQ ID NO: 8169 - RNA, 20 nt, synthetic construct
  source 1..20: mol_type = other RNA
ttcctcaagacatttgggga

SEQ ID NO: 8170 - RNA, 20 nt, synthetic construct
  source 1..20: mol_type = other RNA
ttttttcctcaagacatttg

SEQ ID NO: 8171 - RNA, 20 nt, synthetic construct
  source 1..20: mol_type = other RNA
cttttttcctcaagacattt

SEQ ID NO: 8172 - RNA, 20 nt, synthetic construct
  source 1..20: mol_type = other RNA
gcttttttcctcaagacatt

SEQ ID NO: 8173 - RNA, 20 nt, synthetic construct
  source 1..20: mol_type = other RNA
agccatctgcctccttgttc

SEQ ID NO: 8174 - RNA, 20 nt, synthetic construct
  source 1..20: mol_type = other RNA
gtcctgaacaaggaggcaga

SEQ ID NO: 8175 - RNA, 20 nt, synthetic construct
  source 1..20: mol_type = other RNA
ctccttgttcaggacagcca

SEQ ID NO: 8176 - RNA, 20 nt, synthetic construct
  source 1..20: mol_type = other RNA
tccttgttcaggacagccat

SEQ ID NO: 8177 - RNA, 20 nt, synthetic construct
  source 1..20: mol_type = other RNA
ccttgttcaggacagccatg

SEQ ID NO: 8178 - RNA, 20 nt, synthetic construct
  source 1..20: mol_type = other RNA
catggctgtcctgaacaagg

SEQ ID NO: 8179 - RNA, 20 nt, synthetic construct
  source 1..20: mol_type = other RNA
ccccatggctgtcctgaaca

SEQ ID NO: 8180 - RNA, 20 nt, synthetic construct
  source 1..20: mol_type = other RNA
atgagtcttaaatgacccca

SEQ ID NO: 8181 - RNA, 20 nt, synthetic construct
  source 1..20: mol_type = other RNA
caaccttatcctacgctgtg

SEQ ID NO: 8182 - RNA, 20 nt, synthetic construct
  source 1..20: mol_type = other RNA
ggtccacacagcgtaggata

SEQ ID NO: 8183 - RNA, 20 nt, synthetic construct
  source 1..20: mol_type = other RNA
catcttggtccacacagcgt

SEQ ID NO: 8184 - RNA, 20 nt, synthetic construct
  source 1..20: mol_type = other RNA
tgtggaccaagatgaccatc

SEQ ID NO: 8185 - RNA, 20 nt, synthetic construct
  source 1..20: mol_type = other RNA
caggagccagatggtcatct

SEQ ID NO: 8186 - RNA, 20 nt, synthetic construct
  source 1..20: mol_type = other RNA
tctggctcctgtgattgcag

SEQ ID NO: 8187 - RNA, 20 nt, synthetic construct
  source 1..20: mol_type = other RNA
ctggctcctgtgattgcagt

SEQ ID NO: 8188 - RNA, 20 nt, synthetic construct
  source 1..20: mol_type = other RNA
ctgcaatcacaggagccaga

SEQ ID NO: 8189 - RNA, 20 nt, synthetic construct
  source 1..20: mol_type = other RNA
gtggtccccactgcaatcac

SEQ ID NO: 8190 - RNA, 20 nt, synthetic construct
  source 1..20: mol_type = other RNA
agtggggaccacattgtacc

SEQ ID NO: 8191 - RNA, 20 nt, synthetic construct
  source 1..20: mol_type = other RNA
gtggggaccacattgtacct

SEQ ID NO: 8192 - RNA, 20 nt, synthetic construct
  source 1..20: mol_type = other RNA
attgtacctgggtattacag

SEQ ID NO: 8193 - RNA, 20 nt, synthetic construct
  source 1..20: mol_type = other RNA
tgtaatacccaggtacaatg

SEQ ID NO: 8194 - RNA, 20 nt, synthetic construct
  source 1..20: mol_type = other RNA
gctgcacctctgtaataccc

SEQ ID NO: 8195 - RNA, 20 nt, synthetic construct
  source 1..20: mol_type = other RNA
agctgcagggggaggggaga

SEQ ID NO: 8196 - RNA, 20 nt, synthetic construct
  source 1..20: mol_type = other RNA
ctggacagctgcagggggag

SEQ ID NO: 8197 - RNA, 20 nt, synthetic construct
  source 1..20: mol_type = other RNA
actggacagctgcaggggga

SEQ ID NO: 8198 - RNA, 20 nt, synthetic construct
  source 1..20: mol_type = other RNA
aactggacagctgcaggggg

SEQ ID NO: 8199 - RNA, 20 nt, synthetic construct
  source 1..20: mol_type = other RNA
aggaactggacagctgcagg

SEQ ID NO: 8200 - RNA, 20 nt, synthetic construct
  source 1..20: mol_type = other RNA
caggaactggacagctgcag

SEQ ID NO: 8201 - RNA, 20 nt, synthetic construct
  source 1..20: mol_type = other RNA
ccaggaactggacagctgca

SEQ ID NO: 8202 - RNA, 20 nt, synthetic construct
  source 1..20: mol_type = other RNA
tccaggaactggacagctgc

SEQ ID NO: 8203 - RNA, 20 nt, synthetic construct
  source 1..20: mol_type = other RNA
ttcctggaaaacgtgctccc

SEQ ID NO: 8204 - RNA, 20 nt, synthetic construct
  source 1..20: mol_type = other RNA
ggagcacgttttccaggaac

SEQ ID NO: 8205 - RNA, 20 nt, synthetic construct
  source 1..20: mol_type = other RNA
gtcctgggagcacgttttcc

SEQ ID NO: 8206 - RNA, 20 nt, synthetic construct
  source 1..20: mol_type = other RNA
cacaagcagctgaaggtcct

SEQ ID NO: 8207 - RNA, 20 nt, synthetic construct
  source 1..20: mol_type = other RNA
tcacaagcagctgaaggtcc

SEQ ID NO: 8208 - RNA, 20 nt, synthetic construct
  source 1..20: mol_type = other RNA
ttcagctgcttgtgactaga

SEQ ID NO: 8209 - RNA, 20 nt, synthetic construct
  source 1..20: mol_type = other RNA
agctgcttgtgactagatgg

SEQ ID NO: 8210 - RNA, 20 nt, synthetic construct
  source 1..20: mol_type = other RNA
tttgtggcagagaggattag

SEQ ID NO: 8211 - RNA, 20 nt, synthetic construct
  source 1..20: mol_type = other RNA
ttatgatgtttgtggcagag

SEQ ID NO: 8212 - RNA, 20 nt, synthetic construct
  source 1..20: mol_type = other RNA
cgatctgcttatgatgtttg

SEQ ID NO: 8213 - RNA, 20 nt, synthetic construct
  source 1..20: mol_type = other RNA
cagatcgtataaacgtgaag

SEQ ID NO: 8214 - RNA, 20 nt, synthetic construct
  source 1..20: mol_type = other RNA
aggatgctttttctttaata

SEQ ID NO: 8215 - RNA, 20 nt, synthetic construct
  source 1..20: mol_type = other RNA
gcatcctatgagctatttat

SEQ ID NO: 8216 - RNA, 20 nt, synthetic construct
  source 1..20: mol_type = other RNA
cctatgagctatttattggc

SEQ ID NO: 8217 - RNA, 20 nt, synthetic construct
  source 1..20: mol_type = other RNA
ccagccaataaatagctcat

SEQ ID NO: 8218 - RNA, 20 nt, synthetic construct
  source 1..20: mol_type = other RNA
gctatttattggctggagat

SEQ ID NO: 8219 - RNA, 20 nt, synthetic construct
  source 1..20: mol_type = other RNA
ggtagatgatcctcacacta

SEQ ID NO: 8220 - RNA, 20 nt, synthetic construct
  source 1..20: mol_type = other RNA
catggaaatgccttagtgtg

SEQ ID NO: 8221 - RNA, 20 nt, synthetic construct
  source 1..20: mol_type = other RNA
aaaaaaaaaaaatgaattca

SEQ ID NO: 8222 - RNA, 20 nt, synthetic construct
  source 1..20: mol_type = other RNA
tttttttttttttttgagac

SEQ ID NO: 8223 - RNA, 20 nt, synthetic construct
  source 1..20: mol_type = other RNA
aggatctcactttgtcatcc

SEQ ID NO: 8224 - RNA, 20 nt, synthetic construct
  source 1..20: mol_type = other RNA
tctcactttgtcatccaggc

SEQ ID NO: 8225 - RNA, 20 nt, synthetic construct
  source 1..20: mol_type = other RNA
tcatccaggctggagtgcag

SEQ ID NO: 8226 - RNA, 20 nt, synthetic construct
  source 1..20: mol_type = other RNA
cacaccactgcactccagcc

SEQ ID NO: 8227 - RNA, 20 nt, synthetic construct
  source 1..20: mol_type = other RNA
tcactgtagcctcaacctcc

SEQ ID NO: 8228 - RNA, 20 nt, synthetic construct
  source 1..20: mol_type = other RNA
cactggaaaccaggaggttg

SEQ ID NO: 8229 - RNA, 20 nt, synthetic construct
  source 1..20: mol_type = other RNA
gaggatcactggaaaccagg

SEQ ID NO: 8230 - RNA, 20 nt, synthetic construct
  source 1..20: mol_type = other RNA
tgggaggatcactggaaacc

SEQ ID NO: 8231 - RNA, 20 nt, synthetic construct
  source 1..20: mol_type = other RNA
ttccagtgatcctcccacct

SEQ ID NO: 8232 - RNA, 20 nt, synthetic construct
  source 1..20: mol_type = other RNA
ggccgaggtgggaggatcac

SEQ ID NO: 8233 - RNA, 20 nt, synthetic construct
  source 1..20: mol_type = other RNA
ctttgggaggccgaggtggg

SEQ ID NO: 8234 - RNA, 20 nt, synthetic construct
  source 1..20: mol_type = other RNA
gcactttgggaggccgaggt

SEQ ID NO: 8235 - RNA, 20 nt, synthetic construct
  source 1..20: mol_type = other RNA
agcactttgggaggccgagg

SEQ ID NO: 8236 - RNA, 20 nt, synthetic construct
  source 1..20: mol_type = other RNA
cgcagcactttgggaggccg

SEQ ID NO: 8237 - RNA, 20 nt, synthetic construct
  source 1..20: mol_type = other RNA
tcccaaagtgctgcgattac

SEQ ID NO: 8238 - RNA, 20 nt, synthetic construct
  source 1..20: mol_type = other RNA
tgtaatcgcagcactttggg

SEQ ID NO: 8239 - RNA, 20 nt, synthetic construct
  source 1..20: mol_type = other RNA
gcctgtaatcgcagcacttt

SEQ ID NO: 8240 - RNA, 20 nt, synthetic construct
  source 1..20: mol_type = other RNA
ggcctgtaatcgcagcactt

SEQ ID NO: 8241 - RNA, 20 nt, synthetic construct
  source 1..20: mol_type = other RNA
tgggctgggcacggtggctc

SEQ ID NO: 8242 - RNA, 20 nt, synthetic construct
  source 1..20: mol_type = other RNA
aattcatgggctgggcacgg

SEQ ID NO: 8243 - RNA, 20 nt, synthetic construct
  source 1..20: mol_type = other RNA
ctgaattcatgggctgggca

SEQ ID NO: 8244 - RNA, 20 nt, synthetic construct
  source 1..20: mol_type = other RNA
taaagctgaattcatgggct

SEQ ID NO: 8245 - RNA, 20 nt, synthetic construct
  source 1..20: mol_type = other RNA
ttaaagctgaattcatgggc

SEQ ID NO: 8246 - RNA, 20 nt, synthetic construct
  source 1..20: mol_type = other RNA
agtattaaagctgaattcat

SEQ ID NO: 8247 - RNA, 20 nt, synthetic construct
  source 1..20: mol_type = other RNA
tagtattaaagctgaattca

SEQ ID NO: 8248 - RNA, 20 nt, synthetic construct
  source 1..20: mol_type = other RNA
tatgcaaagtgctgcaaaag

SEQ ID NO: 8249 - RNA, 20 nt, synthetic construct
  source 1..20: mol_type = other RNA
cattttataatgaaaaattc

SEQ ID NO: 8250 - RNA, 20 nt, synthetic construct
  source 1..20: mol_type = other RNA
tttcattataaaatgaatcc

SEQ ID NO: 8251 - RNA, 20 nt, synthetic construct
  source 1..20: mol_type = other RNA
cattataaaatgaatccagg

SEQ ID NO: 8252 - RNA, 20 nt, synthetic construct
  source 1..20: mol_type = other RNA
atttctatattcaaaccacc

SEQ ID NO: 8253 - RNA, 20 nt, synthetic construct
  source 1..20: mol_type = other RNA
aaaaaaactcactatatacc

SEQ ID NO: 8254 - RNA, 20 nt, synthetic construct
  source 1..20: mol_type = other RNA
aagaaagaaagaaaaagtcc

SEQ ID NO: 8255 - RNA, 20 nt, synthetic construct
  source 1..20: mol_type = other RNA
ttctttcttttttttttttt

SEQ ID NO: 8256 - RNA, 20 nt, synthetic construct
  source 1..20: mol_type = other RNA
tgagtcttgctttattgccc

SEQ ID NO: 8257 - RNA, 20 nt, synthetic construct
  source 1..20: mol_type = other RNA
ttgctttattgcccaggctg

SEQ ID NO: 8258 - RNA, 20 nt, synthetic construct
  source 1..20: mol_type = other RNA
ttgcccaggctgaggtgcag

SEQ ID NO: 8259 - RNA, 20 nt, synthetic construct
  source 1..20: mol_type = other RNA
gcaccactgcacctcagcct

SEQ ID NO: 8260 - RNA, 20 nt, synthetic construct
  source 1..20: mol_type = other RNA
agcaccactgcacctcagcc

SEQ ID NO: 8261 - RNA, 20 nt, synthetic construct
  source 1..20: mol_type = other RNA
gaggtgcagtggtgctatct

SEQ ID NO: 8262 - RNA, 20 nt, synthetic construct
  source 1..20: mol_type = other RNA
aacatgggaggcggaggttg

SEQ ID NO: 8263 - RNA, 20 nt, synthetic construct
  source 1..20: mol_type = other RNA
cacttgaacatgggaggcgg

SEQ ID NO: 8264 - RNA, 20 nt, synthetic construct
  source 1..20: mol_type = other RNA
agtcacttgaacatgggagg

SEQ ID NO: 8265 - RNA, 20 nt, synthetic construct
  source 1..20: mol_type = other RNA
gagagtcacttgaacatggg

SEQ ID NO: 8266 - RNA, 20 nt, synthetic construct
  source 1..20: mol_type = other RNA
cacgagagtcacttgaacat

SEQ ID NO: 8267 - RNA, 20 nt, synthetic construct
  source 1..20: mol_type = other RNA
gcacgagagtcacttgaaca

SEQ ID NO: 8268 - RNA, 20 nt, synthetic construct
  source 1..20: mol_type = other RNA
gcttcagcctcccaagtagc

SEQ ID NO: 8269 - RNA, 20 nt, synthetic construct
  source 1..20: mol_type = other RNA
cttcagcctcccaagtagct

SEQ ID NO: 8270 - RNA, 20 nt, synthetic construct
  source 1..20: mol_type = other RNA
tcccaagtagctgggattac

SEQ ID NO: 8271 - RNA, 20 nt, synthetic construct
  source 1..20: mol_type = other RNA
tgtaatcccagctacttggg

SEQ ID NO: 8272 - RNA, 20 nt, synthetic construct
  source 1..20: mol_type = other RNA
acctgtaatcccagctactt

SEQ ID NO: 8273 - RNA, 20 nt, synthetic construct
  source 1..20: mol_type = other RNA
cacctgtaatcccagctact

SEQ ID NO: 8274 - RNA, 20 nt, synthetic construct
  source 1..20: mol_type = other RNA
caggtgcccgccaccacacc

SEQ ID NO: 8275 - RNA, 20 nt, synthetic construct
  source 1..20: mol_type = other RNA
aattagccaggtgtggtggc

SEQ ID NO: 8276 - RNA, 20 nt, synthetic construct
  source 1..20: mol_type = other RNA
aaattagccaggtgtggtgg

SEQ ID NO: 8277 - RNA, 20 nt, synthetic construct
  source 1..20: mol_type = other RNA
caaaaattagccaggtgtgg

SEQ ID NO: 8278 - RNA, 20 nt, synthetic construct
  source 1..20: mol_type = other RNA
ttacaaaaattagccaggtg

SEQ ID NO: 8279 - RNA, 20 nt, synthetic construct
  source 1..20: mol_type = other RNA
taaaattacaaaaattagcc

SEQ ID NO: 8280 - RNA, 20 nt, synthetic construct
  source 1..20: mol_type = other RNA
tttgtaattttaatagagac

SEQ ID NO: 8281 - RNA, 20 nt, synthetic construct
  source 1..20: mol_type = other RNA
atagagaccggttttcacca

SEQ ID NO: 8282 - RNA, 20 nt, synthetic construct
  source 1..20: mol_type = other RNA
gaccggttttcaccatggtg

SEQ ID NO: 8283 - RNA, 20 nt, synthetic construct
  source 1..20: mol_type = other RNA
gttttcaccatggtgtggcc

SEQ ID NO: 8284 - RNA, 20 nt, synthetic construct
  source 1..20: mol_type = other RNA
ggccacaccatggtgaaaac

SEQ ID NO: 8285 - RNA, 20 nt, synthetic construct
  source 1..20: mol_type = other RNA
tcaccatggtgtggccaggc

SEQ ID NO: 8286 - RNA, 20 nt, synthetic construct
  source 1..20: mol_type = other RNA
agaccagcctggccacacca

SEQ ID NO: 8287 - RNA, 20 nt, synthetic construct
  source 1..20: mol_type = other RNA
tcagtagtttgagaccagcc

SEQ ID NO: 8288 - RNA, 20 nt, synthetic construct
  source 1..20: mol_type = other RNA
tgaggcaggcagatcacttg

SEQ ID NO: 8289 - RNA, 20 nt, synthetic construct
  source 1..20: mol_type = other RNA
gcctcagactcccaaagtgc

SEQ ID NO: 8290 - RNA, 20 nt, synthetic construct
  source 1..20: mol_type = other RNA
cctcagactcccaaagtgct

SEQ ID NO: 8291 - RNA, 20 nt, synthetic construct
  source 1..20: mol_type = other RNA
gcactttgggagtctgaggc

SEQ ID NO: 8292 - RNA, 20 nt, synthetic construct
  source 1..20: mol_type = other RNA
cccagcactttgggagtctg

SEQ ID NO: 8293 - RNA, 20 nt, synthetic construct
  source 1..20: mol_type = other RNA
tcccaaagtgctgggattac

SEQ ID NO: 8294 - RNA, 20 nt, synthetic construct
  source 1..20: mol_type = other RNA
gcctgtaatcccagcacttt

SEQ ID NO: 8295 - RNA, 20 nt, synthetic construct
  source 1..20: mol_type = other RNA
ggcctgtaatcccagcactt

SEQ ID NO: 8296 - RNA, 20 nt, synthetic construct
  source 1..20: mol_type = other RNA
acaggcctgagccacccccc

SEQ ID NO: 8297 - RNA, 20 nt, synthetic construct
  source 1..20: mol_type = other RNA
aaaggccaggggggtggctc

SEQ ID NO: 8298 - RNA, 20 nt, synthetic construct
  source 1..20: mol_type = other RNA
aaaaagaaaggccagggggg

SEQ ID NO: 8299 - RNA, 20 nt, synthetic construct
  source 1..20: mol_type = other RNA
ttaaaaaagaaaggccaggg

SEQ ID NO: 8300 - RNA, 20 nt, synthetic construct
  source 1..20: mol_type = other RNA
tttaaaaaagaaaggccagg

SEQ ID NO: 8301 - RNA, 20 nt, synthetic construct
  source 1..20: mol_type = other RNA
ttttaaaaaagaaaggccag

SEQ ID NO: 8302 - RNA, 20 nt, synthetic construct
  source 1..20: mol_type = other RNA
tttttaaaaaagaaaggcca

SEQ ID NO: 8303 - RNA, 20 nt, synthetic construct
  source 1..20: mol_type = other RNA
atttttaaaaaagaaaggcc

SEQ ID NO: 8304 - RNA, 20 nt, synthetic construct
  source 1..20: mol_type = other RNA
actctatttttaaaaaagaa

SEQ ID NO: 8305 - RNA, 20 nt, synthetic construct
  source 1..20: mol_type = other RNA
taaaaatagagttgaaaatt

SEQ ID NO: 8306 - RNA, 20 nt, synthetic construct
  source 1..20: mol_type = other RNA
tttagaactctcaatatact

SEQ ID NO: 8307 - RNA, 20 nt, synthetic construct
  source 1..20: mol_type = other RNA
agagttctaaatccattgtc

SEQ ID NO: 8308 - RNA, 20 nt, synthetic construct
  source 1..20: mol_type = other RNA
cattgtcaggtacatacaac

SEQ ID NO: 8309 - RNA, 20 nt, synthetic construct
  source 1..20: mol_type = other RNA
cagttgtatgtacctgacaa

SEQ ID NO: 8310 - RNA, 20 nt, synthetic construct
  source 1..20: mol_type = other RNA
ggcatgttggcagggtaatc

SEQ ID NO: 8311 - RNA, 20 nt, synthetic construct
  source 1..20: mol_type = other RNA
tatagagaggcatgttggca

SEQ ID NO: 8312 - RNA, 20 nt, synthetic construct
  source 1..20: mol_type = other RNA
gtatagagaggcatgttggc

SEQ ID NO: 8313 - RNA, 20 nt, synthetic construct
  source 1..20: mol_type = other RNA
tggtgtatagagaggcatgt

SEQ ID NO: 8314 - RNA, 20 nt, synthetic construct
  source 1..20: mol_type = other RNA
aatgtaattggtgtatagag

SEQ ID NO: 8315 - RNA, 20 nt, synthetic construct
  source 1..20: mol_type = other RNA
atacaccaattacattctac

SEQ ID NO: 8316 - RNA, 20 nt, synthetic construct
  source 1..20: mol_type = other RNA
tacaccaattacattctact

SEQ ID NO: 8317 - RNA, 20 nt, synthetic construct
  source 1..20: mol_type = other RNA
aactcccagtagaatgtaat

SEQ ID NO: 8318 - RNA, 20 nt, synthetic construct
  source 1..20: mol_type = other RNA
actgggagttgttcaactca

SEQ ID NO: 8319 - RNA, 20 nt, synthetic construct
  source 1..20: mol_type = other RNA
atggcaaggcttaatttaca

SEQ ID NO: 8320 - RNA, 20 nt, synthetic construct
  source 1..20: mol_type = other RNA
tgccatatccattgcagaag

SEQ ID NO: 8321 - RNA, 20 nt, synthetic construct
  source 1..20: mol_type = other RNA
gccatatccattgcagaaga

SEQ ID NO: 8322 - RNA, 20 nt, synthetic construct
  source 1..20: mol_type = other RNA
ccatatccattgcagaagag

SEQ ID NO: 8323 - RNA, 20 nt, synthetic construct
  source 1..20: mol_type = other RNA
cccctcttctgcaatggata

SEQ ID NO: 8324 - RNA, 20 nt, synthetic construct
  source 1..20: mol_type = other RNA
aatgcacccctcttctgcaa

SEQ ID NO: 8325 - RNA, 20 nt, synthetic construct
  source 1..20: mol_type = other RNA
cagaagaggggtgcatttac

SEQ ID NO: 8326 - RNA, 20 nt, synthetic construct
  source 1..20: mol_type = other RNA
agaagaggggtgcatttact

SEQ ID NO: 8327 - RNA, 20 nt, synthetic construct
  source 1..20: mol_type = other RNA
gaggggtgcatttactgggt

SEQ ID NO: 8328 - RNA, 20 nt, synthetic construct
  source 1..20: mol_type = other RNA
tgcatttactgggttggaag

SEQ ID NO: 8329 - RNA, 20 nt, synthetic construct
  source 1..20: mol_type = other RNA
gggttggaagtggtgtcacc

SEQ ID NO: 8330 - RNA, 20 nt, synthetic construct
  source 1..20: mol_type = other RNA
ggtgtcaccaggaccagtca

SEQ ID NO: 8331 - RNA, 20 nt, synthetic construct
  source 1..20: mol_type = other RNA
ggagtggccttgactggtcc

SEQ ID NO: 8332 - RNA, 20 nt, synthetic construct
  source 1..20: mol_type = other RNA
tcaaggccactccttaagaa

SEQ ID NO: 8333 - RNA, 20 nt, synthetic construct
  source 1..20: mol_type = other RNA
tcttaaggagtggccttgac

SEQ ID NO: 8334 - RNA, 20 nt, synthetic construct
  source 1..20: mol_type = other RNA
gctgaacctttcttaaggag

SEQ ID NO: 8335 - RNA, 20 nt, synthetic construct
  source 1..20: mol_type = other RNA
gaaatgctgaacctttctta

SEQ ID NO: 8336 - RNA, 20 nt, synthetic construct
  source 1..20: mol_type = other RNA
aaaggttcagcatttcgtca

SEQ ID NO: 8337 - RNA, 20 nt, synthetic construct
  source 1..20: mol_type = other RNA
tttcgtcatggttttatatc

SEQ ID NO: 8338 - RNA, 20 nt, synthetic construct
  source 1..20: mol_type = other RNA
aaaagttaggaaggcaacaa

SEQ ID NO: 8339 - RNA, 20 nt, synthetic construct
  source 1..20: mol_type = other RNA
atatgtttaaaaagttagga

SEQ ID NO: 8340 - RNA, 20 nt, synthetic construct
  source 1..20: mol_type = other RNA
atgaatatgtttaaaaagtt

SEQ ID NO: 8341 - RNA, 20 nt, synthetic construct
  source 1..20: mol_type = other RNA
tcatctatttctctttcagc

SEQ ID NO: 8342 - RNA, 20 nt, synthetic construct
  source 1..20: mol_type = other RNA
ttcctgtgaaaaactctaag

SEQ ID NO: 8343 - RNA, 20 nt, synthetic construct
  source 1..20: mol_type = other RNA
tcctgtgaaaaactctaagt

SEQ ID NO: 8344 - RNA, 20 nt, synthetic construct
  source 1..20: mol_type = other RNA
tcccacttagagtttttcac

SEQ ID NO: 8345 - RNA, 20 nt, synthetic construct
  source 1..20: mol_type = other RNA
ggaatgtacacttctgagat

SEQ ID NO: 8346 - RNA, 20 nt, synthetic construct
  source 1..20: mol_type = other RNA
tagtgcttaagaaaataacc

SEQ ID NO: 8347 - RNA, 20 nt, synthetic construct
  source 1..20: mol_type = other RNA
taaatagatcgttattttcc

SEQ ID NO: 8348 - RNA, 20 nt, synthetic construct
  source 1..20: mol_type = other RNA
gatctatttagttactatcc

SEQ ID NO: 8349 - RNA, 20 nt, synthetic construct
  source 1..20: mol_type = other RNA
agttactatcctggaagtca

SEQ ID NO: 8350 - RNA, 20 nt, synthetic construct
  source 1..20: mol_type = other RNA
gtatggacaccatgacttcc

SEQ ID NO: 8351 - RNA, 20 nt, synthetic construct
  source 1..20: mol_type = other RNA
tggtgtccatactgctaaag

SEQ ID NO: 8352 - RNA, 20 nt, synthetic construct
  source 1..20: mol_type = other RNA
ggtgtccatactgctaaagt

SEQ ID NO: 8353 - RNA, 20 nt, synthetic construct
  source 1..20: mol_type = other RNA
atagacccactttagcagta

SEQ ID NO: 8354 - RNA, 20 nt, synthetic construct
  source 1..20: mol_type = other RNA
aaagtgggtctattcactga

SEQ ID NO: 8355 - RNA, 20 nt, synthetic construct
  source 1..20: mol_type = other RNA
gtgggtctattcactgatgg

SEQ ID NO: 8356 - RNA, 20 nt, synthetic construct
  source 1..20: mol_type = other RNA
tctattcactgatggaggac

SEQ ID NO: 8357 - RNA, 20 nt, synthetic construct
  source 1..20: mol_type = other RNA
ctgatggaggacaggagagt

SEQ ID NO: 8358 - RNA, 20 nt, synthetic construct
  source 1..20: mol_type = other RNA
tgatggaggacaggagagta

SEQ ID NO: 8359 - RNA, 20 nt, synthetic construct
  source 1..20: mol_type = other RNA
gagtagggataaaaacagac

SEQ ID NO: 8360 - RNA, 20 nt, synthetic construct
  source 1..20: mol_type = other RNA
gataaaaacagacaggatcc

SEQ ID NO: 8361 - RNA, 20 nt, synthetic construct
  source 1..20: mol_type = other RNA
aaaacagacaggatccaggc

SEQ ID NO: 8362 - RNA, 20 nt, synthetic construct
  source 1..20: mol_type = other RNA
aaacagacaggatccaggcc

SEQ ID NO: 8363 - RNA, 20 nt, synthetic construct
  source 1..20: mol_type = other RNA
gacaggatccaggccgggca

SEQ ID NO: 8364 - RNA, 20 nt, synthetic construct
  source 1..20: mol_type = other RNA
aggatccaggccgggcatgg

SEQ ID NO: 8365 - RNA, 20 nt, synthetic construct
  source 1..20: mol_type = other RNA
ttgagccaccatgcccggcc

SEQ ID NO: 8366 - RNA, 20 nt, synthetic construct
  source 1..20: mol_type = other RNA
caggtttgagccaccatgcc

SEQ ID NO: 8367 - RNA, 20 nt, synthetic construct
  source 1..20: mol_type = other RNA
ctcaaacctgtaatcccagt

SEQ ID NO: 8368 - RNA, 20 nt, synthetic construct
  source 1..20: mol_type = other RNA
cctgtaatcccagtaggctg

SEQ ID NO: 8369 - RNA, 20 nt, synthetic construct
  source 1..20: mol_type = other RNA
ctgtaatcccagtaggctgt

SEQ ID NO: 8370 - RNA, 20 nt, synthetic construct
  source 1..20: mol_type = other RNA
taatcccagtaggctgtggg

SEQ ID NO: 8371 - RNA, 20 nt, synthetic construct
  source 1..20: mol_type = other RNA
ccacagcctactgggattac

SEQ ID NO: 8372 - RNA, 20 nt, synthetic construct
  source 1..20: mol_type = other RNA
tcccagtaggctgtgggagg

SEQ ID NO: 8373 - RNA, 20 nt, synthetic construct
  source 1..20: mol_type = other RNA
cagtaggctgtgggaggcgg

SEQ ID NO: 8374 - RNA, 20 nt, synthetic construct
  source 1..20: mol_type = other RNA
taggctgtgggaggcggagg

SEQ ID NO: 8375 - RNA, 20 nt, synthetic construct
  source 1..20: mol_type = other RNA
ctccgcctcccacagcctac

SEQ ID NO: 8376 - RNA, 20 nt, synthetic construct
  source 1..20: mol_type = other RNA
ctgtgggaggcggaggcggg

SEQ ID NO: 8377 - RNA, 20 nt, synthetic construct
  source 1..20: mol_type = other RNA
gcggaggcgggcggatcatg

SEQ ID NO: 8378 - RNA, 20 nt, synthetic construct
  source 1..20: mol_type = other RNA
ggcgggcggatcatgaggtc

SEQ ID NO: 8379 - RNA, 20 nt, synthetic construct
  source 1..20: mol_type = other RNA
tcaggagatcgagaccatcc

SEQ ID NO: 8380 - RNA, 20 nt, synthetic construct
  source 1..20: mol_type = other RNA
tttcactgtgttagccagga

SEQ ID NO: 8381 - RNA, 20 nt, synthetic construct
  source 1..20: mol_type = other RNA
agggtttcactgtgttagcc

SEQ ID NO: 8382 - RNA, 20 nt, synthetic construct
  source 1..20: mol_type = other RNA
ttgtatttttagtggagaca

SEQ ID NO: 8383 - RNA, 20 nt, synthetic construct
  source 1..20: mol_type = other RNA
tttgtatttttagtggagac

SEQ ID NO: 8384 - RNA, 20 nt, synthetic construct
  source 1..20: mol_type = other RNA
aattttttttgtatttttag

SEQ ID NO: 8385 - RNA, 20 nt, synthetic construct
  source 1..20: mol_type = other RNA
aaaatacaaaaaaaattagc

SEQ ID NO: 8386 - RNA, 20 nt, synthetic construct
  source 1..20: mol_type = other RNA
aaatacaaaaaaaattagcc

SEQ ID NO: 8387 - RNA, 20 nt, synthetic construct
  source 1..20: mol_type = other RNA
caaaaaaaattagccgggct

SEQ ID NO: 8388 - RNA, 20 nt, synthetic construct
  source 1..20: mol_type = other RNA
aaaaaattagccgggcttgg

SEQ ID NO: 8389 - RNA, 20 nt, synthetic construct
  source 1..20: mol_type = other RNA
aaattagccgggcttggtgg

SEQ ID NO: 8390 - RNA, 20 nt, synthetic construct
  source 1..20: mol_type = other RNA
aattagccgggcttggtggt

SEQ ID NO: 8391 - RNA, 20 nt, synthetic construct
  source 1..20: mol_type = other RNA
ggcttggtggtgggtgcctg

SEQ ID NO: 8392 - RNA, 20 nt, synthetic construct
  source 1..20: mol_type = other RNA
caggcacccaccaccaagcc

SEQ ID NO: 8393 - RNA, 20 nt, synthetic construct
  source 1..20: mol_type = other RNA
gcctgtggtcccagctactc

SEQ ID NO: 8394 - RNA, 20 nt, synthetic construct
  source 1..20: mol_type = other RNA
tgtggtcccagctactcagg

SEQ ID NO: 8395 - RNA, 20 nt, synthetic construct
  source 1..20: mol_type = other RNA
tcctgagtagctgggaccac

SEQ ID NO: 8396 - RNA, 20 nt, synthetic construct
  source 1..20: mol_type = other RNA
gctactcaggaggctgaagc

SEQ ID NO: 8397 - RNA, 20 nt, synthetic construct
  source 1..20: mol_type = other RNA
cttcagcctcctgagtagct

SEQ ID NO: 8398 - RNA, 20 nt, synthetic construct
  source 1..20: mol_type = other RNA
gcttcagcctcctgagtagc

SEQ ID NO: 8399 - RNA, 20 nt, synthetic construct
  source 1..20: mol_type = other RNA
aggaggctgaagcaggagaa

SEQ ID NO: 8400 - RNA, 20 nt, synthetic construct
  source 1..20: mol_type = other RNA
caggagaatggcatgaaccc

SEQ ID NO: 8401 - RNA, 20 nt, synthetic construct
  source 1..20: mol_type = other RNA
gagaatggcatgaacccagg

SEQ ID NO: 8402 - RNA, 20 nt, synthetic construct
  source 1..20: mol_type = other RNA
aatggcatgaacccaggagg

SEQ ID NO: 8403 - RNA, 20 nt, synthetic construct
  source 1..20: mol_type = other RNA
ggcatgaacccaggaggtgg

SEQ ID NO: 8404 - RNA, 20 nt, synthetic construct
  source 1..20: mol_type = other RNA
catagcaacctccacctcct

SEQ ID NO: 8405 - RNA, 20 nt, synthetic construct
  source 1..20: mol_type = other RNA
tcatagcaacctccacctcc

SEQ ID NO: 8406 - RNA, 20 nt, synthetic construct
  source 1..20: mol_type = other RNA
ggagtgcagtggcgcaatct

SEQ ID NO: 8407 - RNA, 20 nt, synthetic construct
  source 1..20: mol_type = other RNA
tgcgccactgcactccagcc

SEQ ID NO: 8408 - RNA, 20 nt, synthetic construct
  source 1..20: mol_type = other RNA
gcgccactgcactccagcct

SEQ ID NO: 8409 - RNA, 20 nt, synthetic construct
  source 1..20: mol_type = other RNA
tcgcccaggctggagtgcag

SEQ ID NO: 8410 - RNA, 20 nt, synthetic construct
  source 1..20: mol_type = other RNA
tctcgctgtgtcgcccaggc

SEQ ID NO: 8411 - RNA, 20 nt, synthetic construct
  source 1..20: mol_type = other RNA
ggagtctcgctgtgtcgccc

SEQ ID NO: 8412 - RNA, 20 nt, synthetic construct
  source 1..20: mol_type = other RNA
atctaaaaaagaaagcagac

SEQ ID NO: 8413 - RNA, 20 nt, synthetic construct
  source 1..20: mol_type = other RNA
tgtctgctttcttttttaga

SEQ ID NO: 8414 - RNA, 20 nt, synthetic construct
  source 1..20: mol_type = other RNA
cagaaagtctgcattggact

SEQ ID NO: 8415 - RNA, 20 nt, synthetic construct
  source 1..20: mol_type = other RNA
tcagaaagtctgcattggac

SEQ ID NO: 8416 - RNA, 20 nt, synthetic construct
  source 1..20: mol_type = other RNA
gaaagtcagaaagtctgcat

SEQ ID NO: 8417 - RNA, 20 nt, synthetic construct
  source 1..20: mol_type = other RNA
actcttgactcatctaaaat

SEQ ID NO: 8418 - RNA, 20 nt, synthetic construct
  source 1..20: mol_type = other RNA
tttaattgaaactgtggatc

SEQ ID NO: 8419 - RNA, 20 nt, synthetic construct
  source 1..20: mol_type = other RNA
tgtcattttaattgaaactg

SEQ ID NO: 8420 - RNA, 20 nt, synthetic construct
  source 1..20: mol_type = other RNA
aacaccaaataacactgtga

SEQ ID NO: 8421 - RNA, 20 nt, synthetic construct
  source 1..20: mol_type = other RNA
ttcacagtgttatttggtgt

SEQ ID NO: 8422 - RNA, 20 nt, synthetic construct
  source 1..20: mol_type = other RNA
acttccttcacagtgttatt

SEQ ID NO: 8423 - RNA, 20 nt, synthetic construct
  source 1..20: mol_type = other RNA
ttgaaaacccctaccacttc

SEQ ID NO: 8424 - RNA, 20 nt, synthetic construct
  source 1..20: mol_type = other RNA
gaagtggtaggggttttcaa

SEQ ID NO: 8425 - RNA, 20 nt, synthetic construct
  source 1..20: mol_type = other RNA
gtgtgcacctgaagtggtag

SEQ ID NO: 8426 - RNA, 20 nt, synthetic construct
  source 1..20: mol_type = other RNA
agtgtgcacctgaagtggta

SEQ ID NO: 8427 - RNA, 20 nt, synthetic construct
  source 1..20: mol_type = other RNA
gagtgtgcacctgaagtggt

SEQ ID NO: 8428 - RNA, 20 nt, synthetic construct
  source 1..20: mol_type = other RNA
gagggagtgtgcacctgaag

SEQ ID NO: 8429 - RNA, 20 nt, synthetic construct
  source 1..20: mol_type = other RNA
caggtgcacactccctctcc

SEQ ID NO: 8430 - RNA, 20 nt, synthetic construct
  source 1..20: mol_type = other RNA
gggagtatgagtcctggaga

SEQ ID NO: 8431 - RNA, 20 nt, synthetic construct
  source 1..20: mol_type = other RNA
tgggagtatgagtcctggag

SEQ ID NO: 8432 - RNA, 20 nt, synthetic construct
  source 1..20: mol_type = other RNA
ctacatgggagtatgagtcc

SEQ ID NO: 8433 - RNA, 20 nt, synthetic construct
  source 1..20: mol_type = other RNA
cagaaaggaatagtctacat

SEQ ID NO: 8434 - RNA, 20 nt, synthetic construct
  source 1..20: mol_type = other RNA
tcagaaaggaatagtctaca

SEQ ID NO: 8435 - RNA, 20 nt, synthetic construct
  source 1..20: mol_type = other RNA
agactattcctttctgacca

SEQ ID NO: 8436 - RNA, 20 nt, synthetic construct
  source 1..20: mol_type = other RNA
ttcctttctgaccaaggaac

SEQ ID NO: 8437 - RNA, 20 nt, synthetic construct
  source 1..20: mol_type = other RNA
ctccagttccttggtcagaa

SEQ ID NO: 8438 - RNA, 20 nt, synthetic construct
  source 1..20: mol_type = other RNA
aggaactggagctattctca

SEQ ID NO: 8439 - RNA, 20 nt, synthetic construct
  source 1..20: mol_type = other RNA
tgagaatagctccagttcct

SEQ ID NO: 8440 - RNA, 20 nt, synthetic construct
  source 1..20: mol_type = other RNA
ctggagctattctcatggtc

SEQ ID NO: 8441 - RNA, 20 nt, synthetic construct
  source 1..20: mol_type = other RNA
gctattctcatggtctggaa

SEQ ID NO: 8442 - RNA, 20 nt, synthetic construct
  source 1..20: mol_type = other RNA
ctattctcatggtctggaat

SEQ ID NO: 8443 - RNA, 20 nt, synthetic construct
  source 1..20: mol_type = other RNA
ctttagcaagtaggcaggaa

SEQ ID NO: 8444 - RNA, 20 nt, synthetic construct
  source 1..20: mol_type = other RNA
aaacactttagcaagtaggc

SEQ ID NO: 8445 - RNA, 20 nt, synthetic construct
  source 1..20: mol_type = other RNA
agagaaacactttagcaagt

SEQ ID NO: 8446 - RNA, 20 nt, synthetic construct
  source 1..20: mol_type = other RNA
cttctcagtcccataccctt

SEQ ID NO: 8447 - RNA, 20 nt, synthetic construct
  source 1..20: mol_type = other RNA
acaactaatccaaagggtat

SEQ ID NO: 8448 - RNA, 20 nt, synthetic construct
  source 1..20: mol_type = other RNA
cacaactaatccaaagggta

SEQ ID NO: 8449 - RNA, 20 nt, synthetic construct
  source 1..20: mol_type = other RNA
tggctcacaactaatccaaa

SEQ ID NO: 8450 - RNA, 20 nt, synthetic construct
  source 1..20: mol_type = other RNA
ctggctcacaactaatccaa

SEQ ID NO: 8451 - RNA, 20 nt, synthetic construct
  source 1..20: mol_type = other RNA
catattgcatattgaagagt

SEQ ID NO: 8452 - RNA, 20 nt, synthetic construct
  source 1..20: mol_type = other RNA
caactcttcaatatgcaata

SEQ ID NO: 8453 - RNA, 20 nt, synthetic construct
  source 1..20: mol_type = other RNA
aagatttgactccttctaac

SEQ ID NO: 8454 - RNA, 20 nt, synthetic construct
  source 1..20: mol_type = other RNA
gagcttgggaacctgttaga

SEQ ID NO: 8455 - RNA, 20 nt, synthetic construct
  source 1..20: mol_type = other RNA
attacaggtcaatagagctt

SEQ ID NO: 8456 - RNA, 20 nt, synthetic construct
  source 1..20: mol_type = other RNA
aattacaggtcaatagagct

SEQ ID NO: 8457 - RNA, 20 nt, synthetic construct
  source 1..20: mol_type = other RNA
ttgtatttttttgcaattac

SEQ ID NO: 8458 - RNA, 20 nt, synthetic construct
  source 1..20: mol_type = other RNA
caacagcaacaaagatcctg

SEQ ID NO: 8459 - RNA, 20 nt, synthetic construct
  source 1..20: mol_type = other RNA
aacagcaacaaagatcctga

SEQ ID NO: 8460 - RNA, 20 nt, synthetic construct
  source 1..20: mol_type = other RNA
caggatctttgttgctgttg

SEQ ID NO: 8461 - RNA, 20 nt, synthetic construct
  source 1..20: mol_type = other RNA
tcaggatctttgttgctgtt

SEQ ID NO: 8462 - RNA, 20 nt, synthetic construct
  source 1..20: mol_type = other RNA
ctcaggatctttgttgctgt

SEQ ID NO: 8463 - RNA, 20 nt, synthetic construct
  source 1..20: mol_type = other RNA
tcctgagggagtgacattaa

SEQ ID NO: 8464 - RNA, 20 nt, synthetic construct
  source 1..20: mol_type = other RNA
accattaatgtcactccctc

SEQ ID NO: 8465 - RNA, 20 nt, synthetic construct
  source 1..20: mol_type = other RNA
cattaatggtagaattttta

SEQ ID NO: 8466 - RNA, 20 nt, synthetic construct
  source 1..20: mol_type = other RNA
gtagaatttttaaggtacag

SEQ ID NO: 8467 - RNA, 20 nt, synthetic construct
  source 1..20: mol_type = other RNA
gtacagcggtagcccccaaa

SEQ ID NO: 8468 - RNA, 20 nt, synthetic construct
  source 1..20: mol_type = other RNA
tacagcggtagcccccaaat

SEQ ID NO: 8469 - RNA, 20 nt, synthetic construct
  source 1..20: mol_type = other RNA
aggaaaaatggcccatttgg

SEQ ID NO: 8470 - RNA, 20 nt, synthetic construct
  source 1..20: mol_type = other RNA
aaggaaaaatggcccatttg

SEQ ID NO: 8471 - RNA, 20 nt, synthetic construct
  source 1..20: mol_type = other RNA
gaaggaaaaatggcccattt

SEQ ID NO: 8472 - RNA, 20 nt, synthetic construct
  source 1..20: mol_type = other RNA
cgaaggaaaaatggcccatt

SEQ ID NO: 8473 - RNA, 20 nt, synthetic construct
  source 1..20: mol_type = other RNA
aagattagacgaaggaaaaa

SEQ ID NO: 8474 - RNA, 20 nt, synthetic construct
  source 1..20: mol_type = other RNA
cttcgtctaatcttattgca

SEQ ID NO: 8475 - RNA, 20 nt, synthetic construct
  source 1..20: mol_type = other RNA
catgcaataagattagacga

SEQ ID NO: 8476 - RNA, 20 nt, synthetic construct
  source 1..20: mol_type = other RNA
tggcaaatatagacagcagc

SEQ ID NO: 8477 - RNA, 20 nt, synthetic construct
  source 1..20: mol_type = other RNA
gcattcctgactgagaaccc

SEQ ID NO: 8478 - RNA, 20 nt, synthetic construct
  source 1..20: mol_type = other RNA
ctgactgagaaccctggtga

SEQ ID NO: 8479 - RNA, 20 nt, synthetic construct
  source 1..20: mol_type = other RNA
catcaccagggttctcagtc

SEQ ID NO: 8480 - RNA, 20 nt, synthetic construct
  source 1..20: mol_type = other RNA
gaaccctggtgatggcctga

SEQ ID NO: 8481 - RNA, 20 nt, synthetic construct
  source 1..20: mol_type = other RNA
cttccatcaggccatcacca

SEQ ID NO: 8482 - RNA, 20 nt, synthetic construct
  source 1..20: mol_type = other RNA
gcttccatcaggccatcacc

SEQ ID NO: 8483 - RNA, 20 nt, synthetic construct
  source 1..20: mol_type = other RNA
gtctcatctctgcttccatc

SEQ ID NO: 8484 - RNA, 20 nt, synthetic construct
  source 1..20: mol_type = other RNA
gagactgtctgatccactcc

SEQ ID NO: 8485 - RNA, 20 nt, synthetic construct
  source 1..20: mol_type = other RNA
ctgatccactccaggcagca

SEQ ID NO: 8486 - RNA, 20 nt, synthetic construct
  source 1..20: mol_type = other RNA
ccaggcagcatggtccctaa

SEQ ID NO: 8487 - RNA, 20 nt, synthetic construct
  source 1..20: mol_type = other RNA
caggcagcatggtccctaaa

SEQ ID NO: 8488 - RNA, 20 nt, synthetic construct
  source 1..20: mol_type = other RNA
cctttagggaccatgctgcc

SEQ ID NO: 8489 - RNA, 20 nt, synthetic construct
  source 1..20: mol_type = other RNA
cctaaagggccctctacagc

SEQ ID NO: 8490 - RNA, 20 nt, synthetic construct
  source 1..20: mol_type = other RNA
ctaaagggccctctacagct

SEQ ID NO: 8491 - RNA, 20 nt, synthetic construct
  source 1..20: mol_type = other RNA
cagctgtagagggcccttta

SEQ ID NO: 8492 - RNA, 20 nt, synthetic construct
  source 1..20: mol_type = other RNA
ccagctgtagagggcccttt

SEQ ID NO: 8493 - RNA, 20 nt, synthetic construct
  source 1..20: mol_type = other RNA
ggtaggctcccagctgtaga

SEQ ID NO: 8494 - RNA, 20 nt, synthetic construct
  source 1..20: mol_type = other RNA
gggtaggctcccagctgtag

SEQ ID NO: 8495 - RNA, 20 nt, synthetic construct
  source 1..20: mol_type = other RNA
ctgttattacagaacagggt

SEQ ID NO: 8496 - RNA, 20 nt, synthetic construct
  source 1..20: mol_type = other RNA
tgtgctgttattacagaaca

SEQ ID NO: 8497 - RNA, 20 nt, synthetic construct
  source 1..20: mol_type = other RNA
atgtgctgttattacagaac

SEQ ID NO: 8498 - RNA, 20 nt, synthetic construct
  source 1..20: mol_type = other RNA
atcagcaacctctatcattg

SEQ ID NO: 8499 - RNA, 20 nt, synthetic construct
  source 1..20: mol_type = other RNA
aacctctatcattgtggcaa

SEQ ID NO: 8500 - RNA, 20 nt, synthetic construct
  source 1..20: mol_type = other RNA
taccattgccacaatgatag

SEQ ID NO: 8501 - RNA, 20 nt, synthetic construct
  source 1..20: mol_type = other RNA
attgattgcctttatgtgcc

SEQ ID NO: 8502 - RNA, 20 nt, synthetic construct
  source 1..20: mol_type = other RNA
gcaacatgcctggcacataa

SEQ ID NO: 8503 - RNA, 20 nt, synthetic construct
  source 1..20: mol_type = other RNA
gcattggctggcaacatgcc

SEQ ID NO: 8504 - RNA, 20 nt, synthetic construct
  source 1..20: mol_type = other RNA
catcattggtttgcattggc

SEQ ID NO: 8505 - RNA, 20 nt, synthetic construct
  source 1..20: mol_type = other RNA
tattcatcattggtttgcat

SEQ ID NO: 8506 - RNA, 20 nt, synthetic construct
  source 1..20: mol_type = other RNA
aaccaatgatgaataagaaa

SEQ ID NO: 8507 - RNA, 20 nt, synthetic construct
  source 1..20: mol_type = other RNA
aaccatttcttattcatcat

SEQ ID NO: 8508 - RNA, 20 nt, synthetic construct
  source 1..20: mol_type = other RNA
taagaaatggttcctccctt

SEQ ID NO: 8509 - RNA, 20 nt, synthetic construct
  source 1..20: mol_type = other RNA
aagaaatggttcctccctta

SEQ ID NO: 8510 - RNA, 20 nt, synthetic construct
  source 1..20: mol_type = other RNA
tcccttagggagctccagtc

SEQ ID NO: 8511 - RNA, 20 nt, synthetic construct
  source 1..20: mol_type = other RNA
agactggagctccctaaggg

SEQ ID NO: 8512 - RNA, 20 nt, synthetic construct
  source 1..20: mol_type = other RNA
ttagggagctccagtctgga

SEQ ID NO: 8513 - RNA, 20 nt, synthetic construct
  source 1..20: mol_type = other RNA
tagggagctccagtctggaa

SEQ ID NO: 8514 - RNA, 20 nt, synthetic construct
  source 1..20: mol_type = other RNA
tccagactggagctccctaa

SEQ ID NO: 8515 - RNA, 20 nt, synthetic construct
  source 1..20: mol_type = other RNA
ttccagactggagctcccta

SEQ ID NO: 8516 - RNA, 20 nt, synthetic construct
  source 1..20: mol_type = other RNA
tccagtctggaagggaactc

SEQ ID NO: 8517 - RNA, 20 nt, synthetic construct
  source 1..20: mol_type = other RNA
gcctgagttcccttccagac

SEQ ID NO: 8518 - RNA, 20 nt, synthetic construct
  source 1..20: mol_type = other RNA
ctcactgaattttcttatcc

SEQ ID NO: 8519 - RNA, 20 nt, synthetic construct
  source 1..20: mol_type = other RNA
tccaggcaacaaactgtccc

SEQ ID NO: 8520 - RNA, 20 nt, synthetic construct
  source 1..20: mol_type = other RNA
tcctgggacagtttgttgcc

SEQ ID NO: 8521 - RNA, 20 nt, synthetic construct
  source 1..20: mol_type = other RNA
gaaactgtttaaaagatcct

SEQ ID NO: 8522 - RNA, 20 nt, synthetic construct
  source 1..20: mol_type = other RNA
ggaaactgtttaaaagatcc

SEQ ID NO: 8523 - RNA, 20 nt, synthetic construct
  source 1..20: mol_type = other RNA
gttacatactcattgcactc

SEQ ID NO: 8524 - RNA, 20 nt, synthetic construct
  source 1..20: mol_type = other RNA
ttaaactcagaacaaagaga

SEQ ID NO: 8525 - RNA, 20 nt, synthetic construct
  source 1..20: mol_type = other RNA
cagaacaaagagaaggatct

SEQ ID NO: 8526 - RNA, 20 nt, synthetic construct
  source 1..20: mol_type = other RNA
taggaatgcaatttcctatg

SEQ ID NO: 8527 - RNA, 20 nt, synthetic construct
  source 1..20: mol_type = other RNA
aacacatctcttggccacat

SEQ ID NO: 8528 - RNA, 20 nt, synthetic construct
  source 1..20: mol_type = other RNA
tgtggtaggaacacatctct

SEQ ID NO: 8529 - RNA, 20 nt, synthetic construct
  source 1..20: mol_type = other RNA
tcctaccacaaacgtattcc

SEQ ID NO: 8530 - RNA, 20 nt, synthetic construct
  source 1..20: mol_type = other RNA
gccaggaatacgtttgtggt

SEQ ID NO: 8531 - RNA, 20 nt, synthetic construct
  source 1..20: mol_type = other RNA
aaacgtattcctggcttctg

SEQ ID NO: 8532 - RNA, 20 nt, synthetic construct
  source 1..20: mol_type = other RNA
agaagccaggaatacgtttg

SEQ ID NO: 8533 - RNA, 20 nt, synthetic construct
  source 1..20: mol_type = other RNA
atcaaagtgcctcagaagcc

SEQ ID NO: 8534 - RNA, 20 nt, synthetic construct
  source 1..20: mol_type = other RNA
actattaaaaatggctgcat

SEQ ID NO: 8535 - RNA, 20 nt, synthetic construct
  source 1..20: mol_type = other RNA
tactattaaaaatggctgca

SEQ ID NO: 8536 - RNA, 20 nt, synthetic construct
  source 1..20: mol_type = other RNA
tagctatttactattaaaaa

SEQ ID NO: 8537 - RNA, 20 nt, synthetic construct
  source 1..20: mol_type = other RNA
atagctaaatattcagaaat

SEQ ID NO: 8538 - RNA, 20 nt, synthetic construct
  source 1..20: mol_type = other RNA
tcacaattatttatttgatt

SEQ ID NO: 8539 - RNA, 20 nt, synthetic construct
  source 1..20: mol_type = other RNA
cacaattatttatttgattt

SEQ ID NO: 8540 - RNA, 20 nt, synthetic construct
  source 1..20: mol_type = other RNA
tatttgatttgggtagtgtc

SEQ ID NO: 8541 - RNA, 20 nt, synthetic construct
  source 1..20: mol_type = other RNA
gatttgggtagtgtcaggct

SEQ ID NO: 8542 - RNA, 20 nt, synthetic construct
  source 1..20: mol_type = other RNA
atttgggtagtgtcaggcta

SEQ ID NO: 8543 - RNA, 20 nt, synthetic construct
  source 1..20: mol_type = other RNA
caggctagggaaacactacc

SEQ ID NO: 8544 - RNA, 20 nt, synthetic construct
  source 1..20: mol_type = other RNA
ctcttcttgtcttggtgtcc

SEQ ID NO: 8545 - RNA, 20 nt, synthetic construct
  source 1..20: mol_type = other RNA
agacaagaagagaaatgtcc

SEQ ID NO: 8546 - RNA, 20 nt, synthetic construct
  source 1..20: mol_type = other RNA
ggacatttctcttcttgtct

SEQ ID NO: 8547 - RNA, 20 nt, synthetic construct
  source 1..20: mol_type = other RNA
agaagagaaatgtcccggta

SEQ ID NO: 8548 - RNA, 20 nt, synthetic construct
  source 1..20: mol_type = other RNA
gagaaatgtcccggtatggc

SEQ ID NO: 8549 - RNA, 20 nt, synthetic construct
  source 1..20: mol_type = other RNA
agaaatgtcccggtatggca

SEQ ID NO: 8550 - RNA, 20 nt, synthetic construct
  source 1..20: mol_type = other RNA
gaaatgtcccggtatggcag

SEQ ID NO: 8551 - RNA, 20 nt, synthetic construct
  source 1..20: mol_type = other RNA
ggtatggcaggggccagatg

SEQ ID NO: 8552 - RNA, 20 nt, synthetic construct
  source 1..20: mol_type = other RNA
gtatggcaggggccagatgc

SEQ ID NO: 8553 - RNA, 20 nt, synthetic construct
  source 1..20: mol_type = other RNA
catctggcccctgccatacc

SEQ ID NO: 8554 - RNA, 20 nt, synthetic construct
  source 1..20: mol_type = other RNA
gcatctggcccctgccatac

SEQ ID NO: 8555 - RNA, 20 nt, synthetic construct
  source 1..20: mol_type = other RNA
caggggccagatgcgggaga

SEQ ID NO: 8556 - RNA, 20 nt, synthetic construct
  source 1..20: mol_type = other RNA
gggccagatgcgggagaagg

SEQ ID NO: 8557 - RNA, 20 nt, synthetic construct
  source 1..20: mol_type = other RNA
ggtcctccttctcccgcatc

SEQ ID NO: 8558 - RNA, 20 nt, synthetic construct
  source 1..20: mol_type = other RNA
ccagttttatcaaatgagcc

SEQ ID NO: 8559 - RNA, 20 nt, synthetic construct
  source 1..20: mol_type = other RNA
gttttatcaaatgagccagg

SEQ ID NO: 8560 - RNA, 20 nt, synthetic construct
  source 1..20: mol_type = other RNA
ttttatcaaatgagccaggt

SEQ ID NO: 8561 - RNA, 20 nt, synthetic construct
  source 1..20: mol_type = other RNA
cctggctcatttgataaaac

SEQ ID NO: 8562 - RNA, 20 nt, synthetic construct
  source 1..20: mol_type = other RNA
caaatgagccaggtgggtaa

SEQ ID NO: 8563 - RNA, 20 nt, synthetic construct
  source 1..20: mol_type = other RNA
aaatgagccaggtgggtaat

SEQ ID NO: 8564 - RNA, 20 nt, synthetic construct
  source 1..20: mol_type = other RNA
aggtgggtaatgggagtgag

SEQ ID NO: 8565 - RNA, 20 nt, synthetic construct
  source 1..20: mol_type = other RNA
ggtgggtaatgggagtgagt

SEQ ID NO: 8566 - RNA, 20 nt, synthetic construct
  source 1..20: mol_type = other RNA
actcactcccattacccacc

SEQ ID NO: 8567 - RNA, 20 nt, synthetic construct
  source 1..20: mol_type = other RNA
tgagtgggagcttcaagtca

SEQ ID NO: 8568 - RNA, 20 nt, synthetic construct
  source 1..20: mol_type = other RNA
ttcaagtcatggagaacaga

SEQ ID NO: 8569 - RNA, 20 nt, synthetic construct
  source 1..20: mol_type = other RNA
agtgttctaagaactcagcg

SEQ ID NO: 8570 - RNA, 20 nt, synthetic construct
  source 1..20: mol_type = other RNA
aggacactcttcaagccacg

SEQ ID NO: 8571 - RNA, 20 nt, synthetic construct
  source 1..20: mol_type = other RNA
gttctaggagctcagcctcg

SEQ ID NO: 8572 - RNA, 20 nt, synthetic construct
  source 1..20: mol_type = other RNA
ggctgagctcctagaactct

SEQ ID NO: 8573 - RNA, 20 nt, synthetic construct
  source 1..20: mol_type = other RNA
ctcctagaactctaggagac

SEQ ID NO: 8574 - RNA, 20 nt, synthetic construct
  source 1..20: mol_type = other RNA
ctcctgtctcctagagttct

SEQ ID NO: 8575 - RNA, 20 nt, synthetic construct
  source 1..20: mol_type = other RNA
ctctaggagacaggagctag

SEQ ID NO: 8576 - RNA, 20 nt, synthetic construct
  source 1..20: mol_type = other RNA
ggagacaggagctagaggag

SEQ ID NO: 8577 - RNA, 20 nt, synthetic construct
  source 1..20: mol_type = other RNA
gacaggagctagaggagagg

SEQ ID NO: 8578 - RNA, 20 nt, synthetic construct
  source 1..20: mol_type = other RNA
acaggagctagaggagaggt

SEQ ID NO: 8579 - RNA, 20 nt, synthetic construct
  source 1..20: mol_type = other RNA
gaggagaggtgggctctcac

SEQ ID NO: 8580 - RNA, 20 nt, synthetic construct
  source 1..20: mol_type = other RNA
ggtgggctctcactggcctg

SEQ ID NO: 8581 - RNA, 20 nt, synthetic construct
  source 1..20: mol_type = other RNA
cactggcctgtggaataaag

SEQ ID NO: 8582 - RNA, 20 nt, synthetic construct
  source 1..20: mol_type = other RNA
catcagcctctttattccac

SEQ ID NO: 8583 - RNA, 20 nt, synthetic construct
  source 1..20: mol_type = other RNA
ctgatgaaccttcccaagcg

SEQ ID NO: 8584 - RNA, 20 nt, synthetic construct
  source 1..20: mol_type = other RNA
tgatgaaccttcccaagcga

SEQ ID NO: 8585 - RNA, 20 nt, synthetic construct
  source 1..20: mol_type = other RNA
tatgagaccctcgcttggga

SEQ ID NO: 8586 - RNA, 20 nt, synthetic construct
  source 1..20: mol_type = other RNA
caagcgagggtctcataagc

SEQ ID NO: 8587 - RNA, 20 nt, synthetic construct
  source 1..20: mol_type = other RNA
aagcgagggtctcataagca

SEQ ID NO: 8588 - RNA, 20 nt, synthetic construct
  source 1..20: mol_type = other RNA
tgcttatgagaccctcgctt

SEQ ID NO: 8589 - RNA, 20 nt, synthetic construct
  source 1..20: mol_type = other RNA
ctgcttatgagaccctcgct

SEQ ID NO: 8590 - RNA, 20 nt, synthetic construct
  source 1..20: mol_type = other RNA
cataagcagggaggaaagta

SEQ ID NO: 8591 - RNA, 20 nt, synthetic construct
  source 1..20: mol_type = other RNA
ataagcagggaggaaagtat

SEQ ID NO: 8592 - RNA, 20 nt, synthetic construct
  source 1..20: mol_type = other RNA
taagcagggaggaaagtatg

SEQ ID NO: 8593 - RNA, 20 nt, synthetic construct
  source 1..20: mol_type = other RNA
gaggaaagtatggggcttag

SEQ ID NO: 8594 - RNA, 20 nt, synthetic construct
  source 1..20: mol_type = other RNA
aggaaagtatggggcttaga

SEQ ID NO: 8595 - RNA, 20 nt, synthetic construct
  source 1..20: mol_type = other RNA
tggggcttagagggagaatc

SEQ ID NO: 8596 - RNA, 20 nt, synthetic construct
  source 1..20: mol_type = other RNA
gcttagagggagaatcaggc

SEQ ID NO: 8597 - RNA, 20 nt, synthetic construct
  source 1..20: mol_type = other RNA
tagagggagaatcaggctgg

SEQ ID NO: 8598 - RNA, 20 nt, synthetic construct
  source 1..20: mol_type = other RNA
tataaataacaacagctgac

SEQ ID NO: 8599 - RNA, 20 nt, synthetic construct
  source 1..20: mol_type = other RNA
aagttaccaagagaacacag

SEQ ID NO: 8600 - RNA, 20 nt, synthetic construct
  source 1..20: mol_type = other RNA
agttaccaagagaacacaga

SEQ ID NO: 8601 - RNA, 20 nt, synthetic construct
  source 1..20: mol_type = other RNA
gagaaccctctgtgttctct

SEQ ID NO: 8602 - RNA, 20 nt, synthetic construct
  source 1..20: mol_type = other RNA
gtccagttttccttgtcctt

SEQ ID NO: 8603 - RNA, 20 nt, synthetic construct
  source 1..20: mol_type = other RNA
aggacaaggaaaactggaca

SEQ ID NO: 8604 - RNA, 20 nt, synthetic construct
  source 1..20: mol_type = other RNA
atcctaaggacaaggaaaac

SEQ ID NO: 8605 - RNA, 20 nt, synthetic construct
  source 1..20: mol_type = other RNA
gctgtgagatcctaaggaca

SEQ ID NO: 8606 - RNA, 20 nt, synthetic construct
  source 1..20: mol_type = other RNA
cattctgctgtgagatccta

SEQ ID NO: 8607 - RNA, 20 nt, synthetic construct
  source 1..20: mol_type = other RNA
aggtgtattcattgtgacaa

SEQ ID NO: 8608 - RNA, 20 nt, synthetic construct
  source 1..20: mol_type = other RNA
ttacgttatcatagcaatat

SEQ ID NO: 8609 - RNA, 20 nt, synthetic construct
  source 1..20: mol_type = other RNA
taacgtaagtccatttgaaa

SEQ ID NO: 8610 - RNA, 20 nt, synthetic construct
  source 1..20: mol_type = other RNA
cagcaagactccatttcaaa

SEQ ID NO: 8611 - RNA, 20 nt, synthetic construct
  source 1..20: mol_type = other RNA
atggagtcttgctgtcaccc

SEQ ID NO: 8612 - RNA, 20 nt, synthetic construct
  source 1..20: mol_type = other RNA
agtcttgctgtcacccaggc

SEQ ID NO: 8613 - RNA, 20 nt, synthetic construct
  source 1..20: mol_type = other RNA
tcacccaggctggagtgcag

SEQ ID NO: 8614 - RNA, 20 nt, synthetic construct
  source 1..20: mol_type = other RNA
acgccgctgcactccagcct

SEQ ID NO: 8615 - RNA, 20 nt, synthetic construct
  source 1..20: mol_type = other RNA
cacgccgctgcactccagcc

SEQ ID NO: 8616 - RNA, 20 nt, synthetic construct
  source 1..20: mol_type = other RNA
tactgcgacctccgcctccc

SEQ ID NO: 8617 - RNA, 20 nt, synthetic construct
  source 1..20: mol_type = other RNA
agcttgaacctgggaggcgg

SEQ ID NO: 8618 - RNA, 20 nt, synthetic construct
  source 1..20: mol_type = other RNA
aacagcttgaacctgggagg

SEQ ID NO: 8619 - RNA, 20 nt, synthetic construct
  source 1..20: mol_type = other RNA
gagaacagcttgaacctggg

SEQ ID NO: 8620 - RNA, 20 nt, synthetic construct
  source 1..20: mol_type = other RNA
caggagaacagcttgaacct

SEQ ID NO: 8621 - RNA, 20 nt, synthetic construct
  source 1..20: mol_type = other RNA
gcaggagaacagcttgaacc

SEQ ID NO: 8622 - RNA, 20 nt, synthetic construct
  source 1..20: mol_type = other RNA
gcctcagcttcctgagtagc

SEQ ID NO: 8623 - RNA, 20 nt, synthetic construct
  source 1..20: mol_type = other RNA
gctactcaggaagctgaggc

SEQ ID NO: 8624 - RNA, 20 nt, synthetic construct
  source 1..20: mol_type = other RNA
tccagctactcaggaagctg

SEQ ID NO: 8625 - RNA, 20 nt, synthetic construct
  source 1..20: mol_type = other RNA
tcctgagtagctggaactac

SEQ ID NO: 8626 - RNA, 20 nt, synthetic construct
  source 1..20: mol_type = other RNA
acctgtagttccagctactc

SEQ ID NO: 8627 - RNA, 20 nt, synthetic construct
  source 1..20: mol_type = other RNA
caggtgcccgccaccacgcc

SEQ ID NO: 8628 - RNA, 20 nt, synthetic construct
  source 1..20: mol_type = other RNA
aattagccgggcgtggtggc

SEQ ID NO: 8629 - RNA, 20 nt, synthetic construct
  source 1..20: mol_type = other RNA
aaattagccgggcgtggtgg

SEQ ID NO: 8630 - RNA, 20 nt, synthetic construct
  source 1..20: mol_type = other RNA
aaaaaattagccgggcgtgg

SEQ ID NO: 8631 - RNA, 20 nt, synthetic construct
  source 1..20: mol_type = other RNA
tacaaaaaattagccgggcg

SEQ ID NO: 8632 - RNA, 20 nt, synthetic construct
  source 1..20: mol_type = other RNA
aaaaatacaaaaaattagcc

SEQ ID NO: 8633 - RNA, 20 nt, synthetic construct
  source 1..20: mol_type = other RNA
taaaaatacaaaaaattagc

SEQ ID NO: 8634 - RNA, 20 nt, synthetic construct
  source 1..20: mol_type = other RNA
tttgtatttttagtagagac

SEQ ID NO: 8635 - RNA, 20 nt, synthetic construct
  source 1..20: mol_type = other RNA
ttgtatttttagtagagaca

SEQ ID NO: 8636 - RNA, 20 nt, synthetic construct
  source 1..20: mol_type = other RNA
agggtttcaccatgttagcc

SEQ ID NO: 8637 - RNA, 20 nt, synthetic construct
  source 1..20: mol_type = other RNA
tttcaccatgttagccagga

SEQ ID NO: 8638 - RNA, 20 nt, synthetic construct
  source 1..20: mol_type = other RNA
caagaccatcctggctaaca

SEQ ID NO: 8639 - RNA, 20 nt, synthetic construct
  source 1..20: mol_type = other RNA
tcaggagatcaagaccatcc

SEQ ID NO: 8640 - RNA, 20 nt, synthetic construct
  source 1..20: mol_type = other RNA
acctcgtgatccgcccgcct

SEQ ID NO: 8641 - RNA, 20 nt, synthetic construct
  source 1..20: mol_type = other RNA
ggcgggcggatcacgaggtc

SEQ ID NO: 8642 - RNA, 20 nt, synthetic construct
  source 1..20: mol_type = other RNA
gccgaggcgggcggatcacg

SEQ ID NO: 8643 - RNA, 20 nt, synthetic construct
  source 1..20: mol_type = other RNA
ttttgggaggccgaggcggg

SEQ ID NO: 8644 - RNA, 20 nt, synthetic construct
  source 1..20: mol_type = other RNA
gcctcggcctcccaaaatgc

SEQ ID NO: 8645 - RNA, 20 nt, synthetic construct
  source 1..20: mol_type = other RNA
cctcggcctcccaaaatgct

SEQ ID NO: 8646 - RNA, 20 nt, synthetic construct
  source 1..20: mol_type = other RNA
gcattttgggaggccgaggc

SEQ ID NO: 8647 - RNA, 20 nt, synthetic construct
  source 1..20: mol_type = other RNA
agcattttgggaggccgagg

SEQ ID NO: 8648 - RNA, 20 nt, synthetic construct
  source 1..20: mol_type = other RNA
cccagcattttgggaggccg

SEQ ID NO: 8649 - RNA, 20 nt, synthetic construct
  source 1..20: mol_type = other RNA
tcccaaaatgctgggattac

SEQ ID NO: 8650 - RNA, 20 nt, synthetic construct
  source 1..20: mol_type = other RNA
tgtaatcccagcattttggg

SEQ ID NO: 8651 - RNA, 20 nt, synthetic construct
  source 1..20: mol_type = other RNA
acctgtaatcccagcatttt

SEQ ID NO: 8652 - RNA, 20 nt, synthetic construct
  source 1..20: mol_type = other RNA
cacctgtaatcccagcattt

SEQ ID NO: 8653 - RNA, 20 nt, synthetic construct
  source 1..20: mol_type = other RNA
caggtgtgagccactgcgcc

SEQ ID NO: 8654 - RNA, 20 nt, synthetic construct
  source 1..20: mol_type = other RNA
atgactggggccgggcgcag

SEQ ID NO: 8655 - RNA, 20 nt, synthetic construct
  source 1..20: mol_type = other RNA
agaaataaatgactggggcc

SEQ ID NO: 8656 - RNA, 20 nt, synthetic construct
  source 1..20: mol_type = other RNA
tagaaataaatgactggggc

SEQ ID NO: 8657 - RNA, 20 nt, synthetic construct
  source 1..20: mol_type = other RNA
ctgatagaaataaatgactg

SEQ ID NO: 8658 - RNA, 20 nt, synthetic construct
  source 1..20: mol_type = other RNA
actgatagaaataaatgact

SEQ ID NO: 8659 - RNA, 20 nt, synthetic construct
  source 1..20: mol_type = other RNA
tactgatagaaataaatgac

SEQ ID NO: 8660 - RNA, 20 nt, synthetic construct
  source 1..20: mol_type = other RNA
tcttgcatgctttcttgctt

SEQ ID NO: 8661 - RNA, 20 nt, synthetic construct
  source 1..20: mol_type = other RNA
caggaacagttgactagtat

SEQ ID NO: 8662 - RNA, 20 nt, synthetic construct
  source 1..20: mol_type = other RNA
ctgttcctgaatcacatata

SEQ ID NO: 8663 - RNA, 20 nt, synthetic construct
  source 1..20: mol_type = other RNA
tagtaccttatatgtgattc

SEQ ID NO: 8664 - RNA, 20 nt, synthetic construct
  source 1..20: mol_type = other RNA
tataaggtactacactatag

SEQ ID NO: 8665 - RNA, 20 nt, synthetic construct
  source 1..20: mol_type = other RNA
gtactacactatagtggtgc

SEQ ID NO: 8666 - RNA, 20 nt, synthetic construct
  source 1..20: mol_type = other RNA
gcactctgtacatacagcaa

SEQ ID NO: 8667 - RNA, 20 nt, synthetic construct
  source 1..20: mol_type = other RNA
cactctgtacatacagcaaa

SEQ ID NO: 8668 - RNA, 20 nt, synthetic construct
  source 1..20: mol_type = other RNA
actctgtacatacagcaaag

SEQ ID NO: 8669 - RNA, 20 nt, synthetic construct
  source 1..20: mol_type = other RNA
gaattaccatgtgctgccca

SEQ ID NO: 8670 - RNA, 20 nt, synthetic construct
  source 1..20: mol_type = other RNA
tgtgctgcccatggtagtga

SEQ ID NO: 8671 - RNA, 20 nt, synthetic construct
  source 1..20: mol_type = other RNA
tcactaccatgggcagcaca

SEQ ID NO: 8672 - RNA, 20 nt, synthetic construct
  source 1..20: mol_type = other RNA
tttgtgtccatcactaccat

SEQ ID NO: 8673 - RNA, 20 nt, synthetic construct
  source 1..20: mol_type = other RNA
atttgtgtccatcactacca

SEQ ID NO: 8674 - RNA, 20 nt, synthetic construct
  source 1..20: mol_type = other RNA
tagtgatggacacaaatcaa

SEQ ID NO: 8675 - RNA, 20 nt, synthetic construct
  source 1..20: mol_type = other RNA
ttatcattacctgtgcaaag

SEQ ID NO: 8676 - RNA, 20 nt, synthetic construct
  source 1..20: mol_type = other RNA
gtgcaaagtggttaaaattc

SEQ ID NO: 8677 - RNA, 20 nt, synthetic construct
  source 1..20: mol_type = other RNA
gaattttaaccactttgcac

SEQ ID NO: 8678 - RNA, 20 nt, synthetic construct
  source 1..20: mol_type = other RNA
tgggactgaaaatgtctttt

SEQ ID NO: 8679 - RNA, 20 nt, synthetic construct
  source 1..20: mol_type = other RNA
aagcatctgattgcattgtt

SEQ ID NO: 8680 - RNA, 20 nt, synthetic construct
  source 1..20: mol_type = other RNA
caagcatctgattgcattgt

SEQ ID NO: 8681 - RNA, 20 nt, synthetic construct
  source 1..20: mol_type = other RNA
ggaaagtatactgcttttgc

SEQ ID NO: 8682 - RNA, 20 nt, synthetic construct
  source 1..20: mol_type = other RNA
cagtatactttccaaattat

SEQ ID NO: 8683 - RNA, 20 nt, synthetic construct
  source 1..20: mol_type = other RNA
atatgcagatacctataatt

SEQ ID NO: 8684 - RNA, 20 nt, synthetic construct
  source 1..20: mol_type = other RNA
cacatataccttaaaactac

SEQ ID NO: 8685 - RNA, 20 nt, synthetic construct
  source 1..20: mol_type = other RNA
acatataccttaaaactact

SEQ ID NO: 8686 - RNA, 20 nt, synthetic construct
  source 1..20: mol_type = other RNA
catataccttaaaactactg

SEQ ID NO: 8687 - RNA, 20 nt, synthetic construct
  source 1..20: mol_type = other RNA
atataccttaaaactactgg

SEQ ID NO: 8688 - RNA, 20 nt, synthetic construct
  source 1..20: mol_type = other RNA
gaatgcccccagtagtttta

SEQ ID NO: 8689 - RNA, 20 nt, synthetic construct
  source 1..20: mol_type = other RNA
cattcaattgccaaatcaaa

SEQ ID NO: 8690 - RNA, 20 nt, synthetic construct
  source 1..20: mol_type = other RNA
gccaaatcaaatggacacct

SEQ ID NO: 8691 - RNA, 20 nt, synthetic construct
  source 1..20: mol_type = other RNA
accaaggtgtccatttgatt

SEQ ID NO: 8692 - RNA, 20 nt, synthetic construct
  source 1..20: mol_type = other RNA
cttggtctccttgtcttgct

SEQ ID NO: 8693 - RNA, 20 nt, synthetic construct
  source 1..20: mol_type = other RNA
caagcaagacaaggagacca

SEQ ID NO: 8694 - RNA, 20 nt, synthetic construct
  source 1..20: mol_type = other RNA
cagagtgaccaagcaagaca

SEQ ID NO: 8695 - RNA, 20 nt, synthetic construct
  source 1..20: mol_type = other RNA
gcacaagaacagctcaatga

SEQ ID NO: 8696 - RNA, 20 nt, synthetic construct
  source 1..20: mol_type = other RNA
tgcagcttctctgattctcg

SEQ ID NO: 8697 - RNA, 20 nt, synthetic construct
  source 1..20: mol_type = other RNA
ttgatgattctacccctttc

SEQ ID NO: 8698 - RNA, 20 nt, synthetic construct
  source 1..20: mol_type = other RNA
gaaaggggtagaatcatcaa

SEQ ID NO: 8699 - RNA, 20 nt, synthetic construct
  source 1..20: mol_type = other RNA
tctgaagggtggccagaaag

SEQ ID NO: 8700 - RNA, 20 nt, synthetic construct
  source 1..20: mol_type = other RNA
ctctgaagggtggccagaaa

SEQ ID NO: 8701 - RNA, 20 nt, synthetic construct
  source 1..20: mol_type = other RNA
gctctgaagggtggccagaa

SEQ ID NO: 8702 - RNA, 20 nt, synthetic construct
  source 1..20: mol_type = other RNA
gtgacagcagctctgaaggg

SEQ ID NO: 8703 - RNA, 20 nt, synthetic construct
  source 1..20: mol_type = other RNA
ttcagagctgctgtcaccct

SEQ ID NO: 8704 - RNA, 20 nt, synthetic construct
  source 1..20: mol_type = other RNA
agggtgacagcagctctgaa

SEQ ID NO: 8705 - RNA, 20 nt, synthetic construct
  source 1..20: mol_type = other RNA
tagggtgacagcagctctga

SEQ ID NO: 8706 - RNA, 20 nt, synthetic construct
  source 1..20: mol_type = other RNA
aaaactgaggctggatccta

SEQ ID NO: 8707 - RNA, 20 nt, synthetic construct
  source 1..20: mol_type = other RNA
gaaaactgaggctggatcct

SEQ ID NO: 8708 - RNA, 20 nt, synthetic construct
  source 1..20: mol_type = other RNA
ccagcctcagttttcttctg

SEQ ID NO: 8709 - RNA, 20 nt, synthetic construct
  source 1..20: mol_type = other RNA
cctcagaagaaaactgaggc

SEQ ID NO: 8710 - RNA, 20 nt, synthetic construct
  source 1..20: mol_type = other RNA
gagacctcagaagaaaactg

SEQ ID NO: 8711 - RNA, 20 nt, synthetic construct
  source 1..20: mol_type = other RNA
gtcatggttgggagtggatg

SEQ ID NO: 8712 - RNA, 20 nt, synthetic construct
  source 1..20: mol_type = other RNA
atggatgtcatggttgggag

SEQ ID NO: 8713 - RNA, 20 nt, synthetic construct
  source 1..20: mol_type = other RNA
cagtcatggatgtcatggtt

SEQ ID NO: 8714 - RNA, 20 nt, synthetic construct
  source 1..20: mol_type = other RNA
gcagtcatggatgtcatggt

SEQ ID NO: 8715 - RNA, 20 nt, synthetic construct
  source 1..20: mol_type = other RNA
ggaagcagtcatggatgtca

SEQ ID NO: 8716 - RNA, 20 nt, synthetic construct
  source 1..20: mol_type = other RNA
gcacttggaggaagcagtca

SEQ ID NO: 8717 - RNA, 20 nt, synthetic construct
  source 1..20: mol_type = other RNA
cctccaagtgccaccccctc

SEQ ID NO: 8718 - RNA, 20 nt, synthetic construct
  source 1..20: mol_type = other RNA
cctgagggggtggcacttgg

SEQ ID NO: 8719 - RNA, 20 nt, synthetic construct
  source 1..20: mol_type = other RNA
tggcctgagggggtggcact

SEQ ID NO: 8720 - RNA, 20 nt, synthetic construct
  source 1..20: mol_type = other RNA
ccccctcaggccactgcgcc

SEQ ID NO: 8721 - RNA, 20 nt, synthetic construct
  source 1..20: mol_type = other RNA
cccctcaggccactgcgcct

SEQ ID NO: 8722 - RNA, 20 nt, synthetic construct
  source 1..20: mol_type = other RNA
ggcgcagtggcctgaggggg

SEQ ID NO: 8723 - RNA, 20 nt, synthetic construct
  source 1..20: mol_type = other RNA
ccaggcgcagtggcctgagg

SEQ ID NO: 8724 - RNA, 20 nt, synthetic construct
  source 1..20: mol_type = other RNA
cccaggcgcagtggcctgag

SEQ ID NO: 8725 - RNA, 20 nt, synthetic construct
  source 1..20: mol_type = other RNA
gcccaggcgcagtggcctga

SEQ ID NO: 8726 - RNA, 20 nt, synthetic construct
  source 1..20: mol_type = other RNA
tgcccaggcgcagtggcctg

SEQ ID NO: 8727 - RNA, 20 nt, synthetic construct
  source 1..20: mol_type = other RNA
gcagagatgcccaggcgcag

SEQ ID NO: 8728 - RNA, 20 nt, synthetic construct
  source 1..20: mol_type = other RNA
gcctgggcatctctgcactg

SEQ ID NO: 8729 - RNA, 20 nt, synthetic construct
  source 1..20: mol_type = other RNA
gccacagtgcagagatgccc

SEQ ID NO: 8730 - RNA, 20 nt, synthetic construct
  source 1..20: mol_type = other RNA
atctctgcactgtggcttcc

SEQ ID NO: 8731 - RNA, 20 nt, synthetic construct
  source 1..20: mol_type = other RNA
tctgcactgtggcttcctgg

SEQ ID NO: 8732 - RNA, 20 nt, synthetic construct
  source 1..20: mol_type = other RNA
aaatatgagctcgagcctcc

SEQ ID NO: 8733 - RNA, 20 nt, synthetic construct
  source 1..20: mol_type = other RNA
cgagctcatattttatctca

SEQ ID NO: 8734 - RNA, 20 nt, synthetic construct
  source 1..20: mol_type = other RNA
gagctcatattttatctcac

SEQ ID NO: 8735 - RNA, 20 nt, synthetic construct
  source 1..20: mol_type = other RNA
cacgggcatcttcagcatct

SEQ ID NO: 8736 - RNA, 20 nt, synthetic construct
  source 1..20: mol_type = other RNA
tcagcatctaggaaaatgcc

SEQ ID NO: 8737 - RNA, 20 nt, synthetic construct
  source 1..20: mol_type = other RNA
ttgtgtggtgattgcatgcc

SEQ ID NO: 8738 - RNA, 20 nt, synthetic construct
  source 1..20: mol_type = other RNA
attgtgtggtgattgcatgc

SEQ ID NO: 8739 - RNA, 20 nt, synthetic construct
  source 1..20: mol_type = other RNA
ctcaacaaacatgtattgtg

SEQ ID NO: 8740 - RNA, 20 nt, synthetic construct
  source 1..20: mol_type = other RNA
ccaataagttaatccctact

SEQ ID NO: 8741 - RNA, 20 nt, synthetic construct
  source 1..20: mol_type = other RNA
ccaagtagggattaacttat

SEQ ID NO: 8742 - RNA, 20 nt, synthetic construct
  source 1..20: mol_type = other RNA
ggtggaggcacatccaagta

SEQ ID NO: 8743 - RNA, 20 nt, synthetic construct
  source 1..20: mol_type = other RNA
aggtggaggcacatccaagt

SEQ ID NO: 8744 - RNA, 20 nt, synthetic construct
  source 1..20: mol_type = other RNA
ggatgtgcctccaccttgac

SEQ ID NO: 8745 - RNA, 20 nt, synthetic construct
  source 1..20: mol_type = other RNA
tttgaggccagtcaaggtgg

SEQ ID NO: 8746 - RNA, 20 nt, synthetic construct
  source 1..20: mol_type = other RNA
tggtttgaggccagtcaagg

SEQ ID NO: 8747 - RNA, 20 nt, synthetic construct
  source 1..20: mol_type = other RNA
ttctggtttgaggccagtca

SEQ ID NO: 8748 - RNA, 20 nt, synthetic construct
  source 1..20: mol_type = other RNA
aggtaataggttctggtttg

SEQ ID NO: 8749 - RNA, 20 nt, synthetic construct
  source 1..20: mol_type = other RNA
gaacctattacctccccacc

SEQ ID NO: 8750 - RNA, 20 nt, synthetic construct
  source 1..20: mol_type = other RNA
ggtggggaggtaataggttc

SEQ ID NO: 8751 - RNA, 20 nt, synthetic construct
  source 1..20: mol_type = other RNA
attccaggtggggaggtaat

SEQ ID NO: 8752 - RNA, 20 nt, synthetic construct
  source 1..20: mol_type = other RNA
tcgttggattccaggtgggg

SEQ ID NO: 8753 - RNA, 20 nt, synthetic construct
  source 1..20: mol_type = other RNA
tgctcgttggattccaggtg

SEQ ID NO: 8754 - RNA, 20 nt, synthetic construct
  source 1..20: mol_type = other RNA
gtgctcgttggattccaggt

SEQ ID NO: 8755 - RNA, 20 nt, synthetic construct
  source 1..20: mol_type = other RNA
ggtgctcgttggattccagg

SEQ ID NO: 8756 - RNA, 20 nt, synthetic construct
  source 1..20: mol_type = other RNA
gaatccaacgagcacccacc

SEQ ID NO: 8757 - RNA, 20 nt, synthetic construct
  source 1..20: mol_type = other RNA
gtgggtgctcgttggattcc

SEQ ID NO: 8758 - RNA, 20 nt, synthetic construct
  source 1..20: mol_type = other RNA
aggaccaggtgggtgctcgt

SEQ ID NO: 8759 - RNA, 20 nt, synthetic construct
  source 1..20: mol_type = other RNA
cccacctggtcctctgcacg

SEQ ID NO: 8760 - RNA, 20 nt, synthetic construct
  source 1..20: mol_type = other RNA
ccacctggtcctctgcacgt

SEQ ID NO: 8761 - RNA, 20 nt, synthetic construct
  source 1..20: mol_type = other RNA
ccacgtgcagaggaccaggt

SEQ ID NO: 8762 - RNA, 20 nt, synthetic construct
  source 1..20: mol_type = other RNA
cccacgtgcagaggaccagg

SEQ ID NO: 8763 - RNA, 20 nt, synthetic construct
  source 1..20: mol_type = other RNA
aaacccacgtgcagaggacc

SEQ ID NO: 8764 - RNA, 20 nt, synthetic construct
  source 1..20: mol_type = other RNA
aagtcaaaacccacgtgcag

SEQ ID NO: 8765 - RNA, 20 nt, synthetic construct
  source 1..20: mol_type = other RNA
tgtctgtagggaggagagag

SEQ ID NO: 8766 - RNA, 20 nt, synthetic construct
  source 1..20: mol_type = other RNA
gagttttgttgtctgtaggg

SEQ ID NO: 8767 - RNA, 20 nt, synthetic construct
  source 1..20: mol_type = other RNA
taggagttttgttgtctgta

SEQ ID NO: 8768 - RNA, 20 nt, synthetic construct
  source 1..20: mol_type = other RNA
ctaggagttttgttgtctgt

SEQ ID NO: 8769 - RNA, 20 nt, synthetic construct
  source 1..20: mol_type = other RNA
gaaataagatggacactgct

SEQ ID NO: 8770 - RNA, 20 nt, synthetic construct
  source 1..20: mol_type = other RNA
cttatttctcaagcttttct

SEQ ID NO: 8771 - RNA, 20 nt, synthetic construct
  source 1..20: mol_type = other RNA
gaaaagcttgagaaataaga

SEQ ID NO: 8772 - RNA, 20 nt, synthetic construct
  source 1..20: mol_type = other RNA
cacaagggatggagaaaggg

SEQ ID NO: 8773 - RNA, 20 nt, synthetic construct
  source 1..20: mol_type = other RNA
cgtcacaagggatggagaaa

SEQ ID NO: 8774 - RNA, 20 nt, synthetic construct
  source 1..20: mol_type = other RNA
gcgtcacaagggatggagaa

SEQ ID NO: 8775 - RNA, 20 nt, synthetic construct
  source 1..20: mol_type = other RNA
catcccttgtgacgctgctt

SEQ ID NO: 8776 - RNA, 20 nt, synthetic construct
  source 1..20: mol_type = other RNA
cgaagcagcgtcacaaggga

SEQ ID NO: 8777 - RNA, 20 nt, synthetic construct
  source 1..20: mol_type = other RNA
aaaccgaagcagcgtcacaa

SEQ ID NO: 8778 - RNA, 20 nt, synthetic construct
  source 1..20: mol_type = other RNA
taaaccgaagcagcgtcaca

SEQ ID NO: 8779 - RNA, 20 nt, synthetic construct
  source 1..20: mol_type = other RNA
gtttacatttcatttctcac

SEQ ID NO: 8780 - RNA, 20 nt, synthetic construct
  source 1..20: mol_type = other RNA
ctctcttcagtcccttctcc

SEQ ID NO: 8781 - RNA, 20 nt, synthetic construct
  source 1..20: mol_type = other RNA
ctggagaagggactgaagag

SEQ ID NO: 8782 - RNA, 20 nt, synthetic construct
  source 1..20: mol_type = other RNA
gggaaatagagcctggagaa

SEQ ID NO: 8783 - RNA, 20 nt, synthetic construct
  source 1..20: mol_type = other RNA
tgggaaatagagcctggaga

SEQ ID NO: 8784 - RNA, 20 nt, synthetic construct
  source 1..20: mol_type = other RNA
gcaaggtgggaaatagagcc

SEQ ID NO: 8785 - RNA, 20 nt, synthetic construct
  source 1..20: mol_type = other RNA
tagggggactgcagcaaggt

SEQ ID NO: 8786 - RNA, 20 nt, synthetic construct
  source 1..20: mol_type = other RNA
atagggggactgcagcaagg

SEQ ID NO: 8787 - RNA, 20 nt, synthetic construct
  source 1..20: mol_type = other RNA
atcatagggggactgcagca

SEQ ID NO: 8788 - RNA, 20 nt, synthetic construct
  source 1..20: mol_type = other RNA
ttaggaatttaaatcatagg

SEQ ID NO: 8789 - RNA, 20 nt, synthetic construct
  source 1..20: mol_type = other RNA
gttaggaatttaaatcatag

SEQ ID NO: 8790 - RNA, 20 nt, synthetic construct
  source 1..20: mol_type = other RNA
tgttaggaatttaaatcata

SEQ ID NO: 8791 - RNA, 20 nt, synthetic construct
  source 1..20: mol_type = other RNA
gtgttaggaatttaaatcat

SEQ ID NO: 8792 - RNA, 20 nt, synthetic construct
  source 1..20: mol_type = other RNA
cctaacactggctgcttctt

SEQ ID NO: 8793 - RNA, 20 nt, synthetic construct
  source 1..20: mol_type = other RNA
ctaacactggctgcttctta

SEQ ID NO: 8794 - RNA, 20 nt, synthetic construct
  source 1..20: mol_type = other RNA
cctaagaagcagccagtgtt

SEQ ID NO: 8795 - RNA, 20 nt, synthetic construct
  source 1..20: mol_type = other RNA
gctgcttcttagggtagaca

SEQ ID NO: 8796 - RNA, 20 nt, synthetic construct
  source 1..20: mol_type = other RNA
agggtagacaaggctcttca

SEQ ID NO: 8797 - RNA, 20 nt, synthetic construct
  source 1..20: mol_type = other RNA
tagacaaggctcttcatggt

SEQ ID NO: 8798 - RNA, 20 nt, synthetic construct
  source 1..20: mol_type = other RNA
agctgactgcagctgctgcc

SEQ ID NO: 8799 - RNA, 20 nt, synthetic construct
  source 1..20: mol_type = other RNA
gcagcagctgcagtcagctg

SEQ ID NO: 8800 - RNA, 20 nt, synthetic construct
  source 1..20: mol_type = other RNA
tgagttacagggctgggacc

SEQ ID NO: 8801 - RNA, 20 nt, synthetic construct
  source 1..20: mol_type = other RNA
ccagccctgtaactcaatac

SEQ ID NO: 8802 - RNA, 20 nt, synthetic construct
  source 1..20: mol_type = other RNA
cagtattgagttacagggct

SEQ ID NO: 8803 - RNA, 20 nt, synthetic construct
  source 1..20: mol_type = other RNA
ccagtattgagttacagggc

SEQ ID NO: 8804 - RNA, 20 nt, synthetic construct
  source 1..20: mol_type = other RNA
cattccagtattgagttaca

SEQ ID NO: 8805 - RNA, 20 nt, synthetic construct
  source 1..20: mol_type = other RNA
tcattccagtattgagttac

SEQ ID NO: 8806 - RNA, 20 nt, synthetic construct
  source 1..20: mol_type = other RNA
agttccacttctctgagtct

SEQ ID NO: 8807 - RNA, 20 nt, synthetic construct
  source 1..20: mol_type = other RNA
cacttctctgagtctcggcc

SEQ ID NO: 8808 - RNA, 20 nt, synthetic construct
  source 1..20: mol_type = other RNA
acttctctgagtctcggcct

SEQ ID NO: 8809 - RNA, 20 nt, synthetic construct
  source 1..20: mol_type = other RNA
caggccgagactcagagaag

SEQ ID NO: 8810 - RNA, 20 nt, synthetic construct
  source 1..20: mol_type = other RNA
tcaggcaggaagggcagccc

SEQ ID NO: 8811 - RNA, 20 nt, synthetic construct
  source 1..20: mol_type = other RNA
agaagggcatcaggcaggaa

SEQ ID NO: 8812 - RNA, 20 nt, synthetic construct
  source 1..20: mol_type = other RNA
gagaagggcatcaggcagga

SEQ ID NO: 8813 - RNA, 20 nt, synthetic construct
  source 1..20: mol_type = other RNA
cagggagaagggcatcaggc

SEQ ID NO: 8814 - RNA, 20 nt, synthetic construct
  source 1..20: mol_type = other RNA
agaacagggagaagggcatc

SEQ ID NO: 8815 - RNA, 20 nt, synthetic construct
  source 1..20: mol_type = other RNA
ataaatgagaacagggagaa

SEQ ID NO: 8816 - RNA, 20 nt, synthetic construct
  source 1..20: mol_type = other RNA
aataaatgagaacagggaga

SEQ ID NO: 8817 - RNA, 20 nt, synthetic construct
  source 1..20: mol_type = other RNA
gtgagtaataaatgagaaca

SEQ ID NO: 8818 - RNA, 20 nt, synthetic construct
  source 1..20: mol_type = other RNA
agtgagtaataaatgagaac

SEQ ID NO: 8819 - RNA, 20 nt, synthetic construct
  source 1..20: mol_type = other RNA
ctcctcaaagaccaccccaa

SEQ ID NO: 8820 - RNA, 20 nt, synthetic construct
  source 1..20: mol_type = other RNA
tcctcaaagaccaccccaaa

SEQ ID NO: 8821 - RNA, 20 nt, synthetic construct
  source 1..20: mol_type = other RNA
gccctttggggtggtctttg

SEQ ID NO: 8822 - RNA, 20 nt, synthetic construct
  source 1..20: mol_type = other RNA
ccccaaagggcacagctttt

SEQ ID NO: 8823 - RNA, 20 nt, synthetic construct
  source 1..20: mol_type = other RNA
aaaagctgtgccctttgggg

SEQ ID NO: 8824 - RNA, 20 nt, synthetic construct
  source 1..20: mol_type = other RNA
ccaaaaagctgtgccctttg

SEQ ID NO: 8825 - RNA, 20 nt, synthetic construct
  source 1..20: mol_type = other RNA
accaaaaagctgtgcccttt

SEQ ID NO: 8826 - RNA, 20 nt, synthetic construct
  source 1..20: mol_type = other RNA
caccaaaaagctgtgccctt

SEQ ID NO: 8827 - RNA, 20 nt, synthetic construct
  source 1..20: mol_type = other RNA
cagcagagggtaattcaata

SEQ ID NO: 8828 - RNA, 20 nt, synthetic construct
  source 1..20: mol_type = other RNA
atagacatgggtacagcaga

SEQ ID NO: 8829 - RNA, 20 nt, synthetic construct
  source 1..20: mol_type = other RNA
aatagacatgggtacagcag

SEQ ID NO: 8830 - RNA, 20 nt, synthetic construct
  source 1..20: mol_type = other RNA
gcaagtgcactaatagacat

SEQ ID NO: 8831 - RNA, 20 nt, synthetic construct
  source 1..20: mol_type = other RNA
ggcaagtgcactaatagaca

SEQ ID NO: 8832 - RNA, 20 nt, synthetic construct
  source 1..20: mol_type = other RNA
gtgcacttgccactccacac

SEQ ID NO: 8833 - RNA, 20 nt, synthetic construct
  source 1..20: mol_type = other RNA
ctaatcattccagtgtggag

SEQ ID NO: 8834 - RNA, 20 nt, synthetic construct
  source 1..20: mol_type = other RNA
gaagactaatcattccagtg

SEQ ID NO: 8835 - RNA, 20 nt, synthetic construct
  source 1..20: mol_type = other RNA
caactgagaagcacatgagt

SEQ ID NO: 8836 - RNA, 20 nt, synthetic construct
  source 1..20: mol_type = other RNA
tggagatacagaaaggagta

SEQ ID NO: 8837 - RNA, 20 nt, synthetic construct
  source 1..20: mol_type = other RNA
tttctgtatctccagtgcct

SEQ ID NO: 8838 - RNA, 20 nt, synthetic construct
  source 1..20: mol_type = other RNA
aaggcactggagatacagaa

SEQ ID NO: 8839 - RNA, 20 nt, synthetic construct
  source 1..20: mol_type = other RNA
ctccagtgccttggagacac

SEQ ID NO: 8840 - RNA, 20 nt, synthetic construct
  source 1..20: mol_type = other RNA
tacctgtgtctccaaggcac

SEQ ID NO: 8841 - RNA, 20 nt, synthetic construct
  source 1..20: mol_type = other RNA
aataaatacctgtgtctcca

SEQ ID NO: 8842 - RNA, 20 nt, synthetic construct
  source 1..20: mol_type = other RNA
agcattcaccccttcaaaat

SEQ ID NO: 8843 - RNA, 20 nt, synthetic construct
  source 1..20: mol_type = other RNA
tcttgtctcctattttgaag

SEQ ID NO: 8844 - RNA, 20 nt, synthetic construct
  source 1..20: mol_type = other RNA
gtcttgtctcctattttgaa

SEQ ID NO: 8845 - RNA, 20 nt, synthetic construct
  source 1..20: mol_type = other RNA
ggtcttgtctcctattttga

SEQ ID NO: 8846 - RNA, 20 nt, synthetic construct
  source 1..20: mol_type = other RNA
ggatcgactgtgctctttgc

SEQ ID NO: 8847 - RNA, 20 nt, synthetic construct
  source 1..20: mol_type = other RNA
agtcgatccacgactccaaa

SEQ ID NO: 8848 - RNA, 20 nt, synthetic construct
  source 1..20: mol_type = other RNA
atccacgactccaaatggaa

SEQ ID NO: 8849 - RNA, 20 nt, synthetic construct
  source 1..20: mol_type = other RNA
ttccattccatttggagtcg

SEQ ID NO: 8850 - RNA, 20 nt, synthetic construct
  source 1..20: mol_type = other RNA
taaatgtattccattccatt

SEQ ID NO: 8851 - RNA, 20 nt, synthetic construct
  source 1..20: mol_type = other RNA
gaatacatttaaaatacatc

SEQ ID NO: 8852 - RNA, 20 nt, synthetic construct
  source 1..20: mol_type = other RNA
catttaaaatacatctggag

SEQ ID NO: 8853 - RNA, 20 nt, synthetic construct
  source 1..20: mol_type = other RNA
atttaaaatacatctggagt

SEQ ID NO: 8854 - RNA, 20 nt, synthetic construct
  source 1..20: mol_type = other RNA
ctttaaaaaacaacacttag

SEQ ID NO: 8855 - RNA, 20 nt, synthetic construct
  source 1..20: mol_type = other RNA
aaaacaacacttagaggcca

SEQ ID NO: 8856 - RNA, 20 nt, synthetic construct
  source 1..20: mol_type = other RNA
caacacttagaggccaaggc

SEQ ID NO: 8857 - RNA, 20 nt, synthetic construct
  source 1..20: mol_type = other RNA
cacttagaggccaaggcagg

SEQ ID NO: 8858 - RNA, 20 nt, synthetic construct
  source 1..20: mol_type = other RNA
caaggcaggtggatcacctg

SEQ ID NO: 8859 - RNA, 20 nt, synthetic construct
  source 1..20: mol_type = other RNA
ctcaggtgatccacctgcct

SEQ ID NO: 8860 - RNA, 20 nt, synthetic construct
  source 1..20: mol_type = other RNA
caggtggatcacctgaggtc

SEQ ID NO: 8861 - RNA, 20 nt, synthetic construct
  source 1..20: mol_type = other RNA
ggtctcgaactcctgacctc

SEQ ID NO: 8862 - RNA, 20 nt, synthetic construct
  source 1..20: mol_type = other RNA
cgagaccagcatgaccaata

SEQ ID NO: 8863 - RNA, 20 nt, synthetic construct
  source 1..20: mol_type = other RNA
tctcaccatattggtcatgc

SEQ ID NO: 8864 - RNA, 20 nt, synthetic construct
  source 1..20: mol_type = other RNA
gagatggggtctcaccatat

SEQ ID NO: 8865 - RNA, 20 nt, synthetic construct
  source 1..20: mol_type = other RNA
ttgtatttttggtagagatg

SEQ ID NO: 8866 - RNA, 20 nt, synthetic construct
  source 1..20: mol_type = other RNA
tttgtatttttggtagagat

SEQ ID NO: 8867 - RNA, 20 nt, synthetic construct
  source 1..20: mol_type = other RNA
ttttgtatttttggtagaga

SEQ ID NO: 8868 - RNA, 20 nt, synthetic construct
  source 1..20: mol_type = other RNA
ccaaaaatacaaaaattagc

SEQ ID NO: 8869 - RNA, 20 nt, synthetic construct
  source 1..20: mol_type = other RNA
caaaaatacaaaaattagct

SEQ ID NO: 8870 - RNA, 20 nt, synthetic construct
  source 1..20: mol_type = other RNA
ccagctaatttttgtatttt

SEQ ID NO: 8871 - RNA, 20 nt, synthetic construct
  source 1..20: mol_type = other RNA
caaaaattagctgggcatga

SEQ ID NO: 8872 - RNA, 20 nt, synthetic construct
  source 1..20: mol_type = other RNA
tgcctgtagtcccagctact

SEQ ID NO: 8873 - RNA, 20 nt, synthetic construct
  source 1..20: mol_type = other RNA
gcctgtagtcccagctactt

SEQ ID NO: 8874 - RNA, 20 nt, synthetic construct
  source 1..20: mol_type = other RNA
tgtagtcccagctacttggg

SEQ ID NO: 8875 - RNA, 20 nt, synthetic construct
  source 1..20: mol_type = other RNA
tcccaagtagctgggactac

SEQ ID NO: 8876 - RNA, 20 nt, synthetic construct
  source 1..20: mol_type = other RNA
gtcccagctacttgggaggc

SEQ ID NO: 8877 - RNA, 20 nt, synthetic construct
  source 1..20: mol_type = other RNA
tcccagctacttgggaggct

SEQ ID NO: 8878 - RNA, 20 nt, synthetic construct
  source 1..20: mol_type = other RNA
gctacttgggaggctgggac

SEQ ID NO: 8879 - RNA, 20 nt, synthetic construct
  source 1..20: mol_type = other RNA
tcccagcctcccaagtagct

SEQ ID NO: 8880 - RNA, 20 nt, synthetic construct
  source 1..20: mol_type = other RNA
gtcccagcctcccaagtagc

SEQ ID NO: 8881 - RNA, 20 nt, synthetic construct
  source 1..20: mol_type = other RNA
acaggagaattgcttgaacc

SEQ ID NO: 8882 - RNA, 20 nt, synthetic construct
  source 1..20: mol_type = other RNA
caggagaattgcttgaacct

SEQ ID NO: 8883 - RNA, 20 nt, synthetic construct
  source 1..20: mol_type = other RNA
gagaattgcttgaacctggg

SEQ ID NO: 8884 - RNA, 20 nt, synthetic construct
  source 1..20: mol_type = other RNA
aattgcttgaacctgggagg

SEQ ID NO: 8885 - RNA, 20 nt, synthetic construct
  source 1..20: mol_type = other RNA
tgcttgaacctgggaggtgg

SEQ ID NO: 8886 - RNA, 20 nt, synthetic construct
  source 1..20: mol_type = other RNA
cactgcaacctccacctccc

SEQ ID NO: 8887 - RNA, 20 nt, synthetic construct
  source 1..20: mol_type = other RNA
ggagtgcagtcgtgtgatct

SEQ ID NO: 8888 - RNA, 20 nt, synthetic construct
  source 1..20: mol_type = other RNA
cacacgactgcactccagcc

SEQ ID NO: 8889 - RNA, 20 nt, synthetic construct
  source 1..20: mol_type = other RNA
acacgactgcactccagcct

SEQ ID NO: 8890 - RNA, 20 nt, synthetic construct
  source 1..20: mol_type = other RNA
tctcgctctgtcacccaggc

SEQ ID NO: 8891 - RNA, 20 nt, synthetic construct
  source 1..20: mol_type = other RNA
agagtctcgctctgtcaccc

SEQ ID NO: 8892 - RNA, 20 nt, synthetic construct
  source 1..20: mol_type = other RNA
gggtttttttgggggtgggg

SEQ ID NO: 8893 - RNA, 20 nt, synthetic construct
  source 1..20: mol_type = other RNA
ggggtttttttgggggtggg

SEQ ID NO: 8894 - RNA, 20 nt, synthetic construct
  source 1..20: mol_type = other RNA
tggggtttttttgggggtgg

SEQ ID NO: 8895 - RNA, 20 nt, synthetic construct
  source 1..20: mol_type = other RNA
gtggggtttttttgggggtg

SEQ ID NO: 8896 - RNA, 20 nt, synthetic construct
  source 1..20: mol_type = other RNA
tgtggggtttttttgggggt

SEQ ID NO: 8897 - RNA, 20 nt, synthetic construct
  source 1..20: mol_type = other RNA
ttgtggggtttttttggggg

SEQ ID NO: 8898 - RNA, 20 nt, synthetic construct
  source 1..20: mol_type = other RNA
gtgttgtggggtttttttgg

SEQ ID NO: 8899 - RNA, 20 nt, synthetic construct
  source 1..20: mol_type = other RNA
ggtgttgtggggtttttttg

SEQ ID NO: 8900 - RNA, 20 nt, synthetic construct
  source 1..20: mol_type = other RNA
aggtgttgtggggttttttt

SEQ ID NO: 8901 - RNA, 20 nt, synthetic construct
  source 1..20: mol_type = other RNA
taggtgttgtggggtttttt

SEQ ID NO: 8902 - RNA, 20 nt, synthetic construct
  source 1..20: mol_type = other RNA
ttataaatttaggtgttgtg

SEQ ID NO: 8903 - RNA, 20 nt, synthetic construct
  source 1..20: mol_type = other RNA
attataaatttaggtgttgt

SEQ ID NO: 8904 - RNA, 20 nt, synthetic construct
  source 1..20: mol_type = other RNA
tattataaatttaggtgttg

SEQ ID NO: 8905 - RNA, 20 nt, synthetic construct
  source 1..20: mol_type = other RNA
attgtggttattataaattt

SEQ ID NO: 8906 - RNA, 20 nt, synthetic construct
  source 1..20: mol_type = other RNA
aataataataataaagattg

SEQ ID NO: 8907 - RNA, 20 nt, synthetic construct
  source 1..20: mol_type = other RNA
acagtctcgctctgtcgccc

SEQ ID NO: 8908 - RNA, 20 nt, synthetic construct
  source 1..20: mol_type = other RNA
tctcgctctgtcgcccaggc

SEQ ID NO: 8909 - RNA, 20 nt, synthetic construct
  source 1..20: mol_type = other RNA
tcgcccaggctggagtgcag

SEQ ID NO: 8910 - RNA, 20 nt, synthetic construct
  source 1..20: mol_type = other RNA
gcgccactgcactccagcct

SEQ ID NO: 8911 - RNA, 20 nt, synthetic construct
  source 1..20: mol_type = other RNA
cgcgccactgcactccagcc

SEQ ID NO: 8912 - RNA, 20 nt, synthetic construct
  source 1..20: mol_type = other RNA
ggagtgcagtggcgcgatct

SEQ ID NO: 8913 - RNA, 20 nt, synthetic construct
  source 1..20: mol_type = other RNA
tcactgcaagctccgcctcc

SEQ ID NO: 8914 - RNA, 20 nt, synthetic construct
  source 1..20: mol_type = other RNA
cactgcaagctccgcctccc

SEQ ID NO: 8915 - RNA, 20 nt, synthetic construct
  source 1..20: mol_type = other RNA
aatggcgtgaacccgggagg

SEQ ID NO: 8916 - RNA, 20 nt, synthetic construct
  source 1..20: mol_type = other RNA
gaaaatggcgtgaacccggg

SEQ ID NO: 8917 - RNA, 20 nt, synthetic construct
  source 1..20: mol_type = other RNA
caggaaaatggcgtgaaccc

SEQ ID NO: 8918 - RNA, 20 nt, synthetic construct
  source 1..20: mol_type = other RNA
gcaggaaaatggcgtgaacc

SEQ ID NO: 8919 - RNA, 20 nt, synthetic construct
  source 1..20: mol_type = other RNA
gggaggctgaggcaggaaaa

SEQ ID NO: 8920 - RNA, 20 nt, synthetic construct
  source 1..20: mol_type = other RNA
gcctcagcctcccgagtagc

SEQ ID NO: 8921 - RNA, 20 nt, synthetic construct
  source 1..20: mol_type = other RNA
cctcagcctcccgagtagct

SEQ ID NO: 8922 - RNA, 20 nt, synthetic construct
  source 1..20: mol_type = other RNA
gctactcgggaggctgaggc

SEQ ID NO: 8923 - RNA, 20 nt, synthetic construct
  source 1..20: mol_type = other RNA
cccagctactcgggaggctg

SEQ ID NO: 8924 - RNA, 20 nt, synthetic construct
  source 1..20: mol_type = other RNA
tcccgagtagctgggactac

SEQ ID NO: 8925 - RNA, 20 nt, synthetic construct
  source 1..20: mol_type = other RNA
tgtagtcccagctactcggg

SEQ ID NO: 8926 - RNA, 20 nt, synthetic construct
  source 1..20: mol_type = other RNA
gcctgtagtcccagctactc

SEQ ID NO: 8927 - RNA, 20 nt, synthetic construct
  source 1..20: mol_type = other RNA
tgcctgtagtcccagctact

SEQ ID NO: 8928 - RNA, 20 nt, synthetic construct
  source 1..20: mol_type = other RNA
caggcacccgccaccacgcc

SEQ ID NO: 8929 - RNA, 20 nt, synthetic construct
  source 1..20: mol_type = other RNA
aattagccgggcgtggtggc

SEQ ID NO: 8930 - RNA, 20 nt, synthetic construct
  source 1..20: mol_type = other RNA
aaattagccgggcgtggtgg

SEQ ID NO: 8931 - RNA, 20 nt, synthetic construct
  source 1..20: mol_type = other RNA
aaaaaattagccgggcgtgg

SEQ ID NO: 8932 - RNA, 20 nt, synthetic construct
  source 1..20: mol_type = other RNA
acaaaaaaattagccgggcg

SEQ ID NO: 8933 - RNA, 20 nt, synthetic construct
  source 1..20: mol_type = other RNA
aaaatacaaaaaaattagcc

SEQ ID NO: 8934 - RNA, 20 nt, synthetic construct
  source 1..20: mol_type = other RNA
aaaaatacaaaaaaattagc

SEQ ID NO: 8935 - RNA, 20 nt, synthetic construct
  source 1..20: mol_type = other RNA
ttttgtatttttagtagaga

SEQ ID NO: 8936 - RNA, 20 nt, synthetic construct
  source 1..20: mol_type = other RNA
tttgtatttttagtagagat

SEQ ID NO: 8937 - RNA, 20 nt, synthetic construct
  source 1..20: mol_type = other RNA
ttgtatttttagtagagatg

SEQ ID NO: 8938 - RNA, 20 nt, synthetic construct
  source 1..20: mol_type = other RNA
ggggtttcaccgtgttagcc

SEQ ID NO: 8939 - RNA, 20 nt, synthetic construct
  source 1..20: mol_type = other RNA
tttcaccgtgttagccagga

SEQ ID NO: 8940 - RNA, 20 nt, synthetic construct
  source 1..20: mol_type = other RNA
cgagaccatcctggctaaca

SEQ ID NO: 8941 - RNA, 20 nt, synthetic construct
  source 1..20: mol_type = other RNA
tcaggagatcgagaccatcc

SEQ ID NO: 8942 - RNA, 20 nt, synthetic construct
  source 1..20: mol_type = other RNA
acctcgtgatccgcccgcct

SEQ ID NO: 8943 - RNA, 20 nt, synthetic construct
  source 1..20: mol_type = other RNA
ggcgggcggatcacgaggtc

SEQ ID NO: 8944 - RNA, 20 nt, synthetic construct
  source 1..20: mol_type = other RNA
gccgaggcgggcggatcacg

SEQ ID NO: 8945 - RNA, 20 nt, synthetic construct
  source 1..20: mol_type = other RNA
ctttgggaggccgaggcggg

SEQ ID NO: 8946 - RNA, 20 nt, synthetic construct
  source 1..20: mol_type = other RNA
gcctcggcctcccaaagtgc

SEQ ID NO: 8947 - RNA, 20 nt, synthetic construct
  source 1..20: mol_type = other RNA
cctcggcctcccaaagtgct

SEQ ID NO: 8948 - RNA, 20 nt, synthetic construct
  source 1..20: mol_type = other RNA
gcactttgggaggccgaggc

SEQ ID NO: 8949 - RNA, 20 nt, synthetic construct
  source 1..20: mol_type = other RNA
agcactttgggaggccgagg

SEQ ID NO: 8950 - RNA, 20 nt, synthetic construct
  source 1..20: mol_type = other RNA
cccagcactttgggaggccg

SEQ ID NO: 8951 - RNA, 20 nt, synthetic construct
  source 1..20: mol_type = other RNA
tcccaaagtgctgggattac

SEQ ID NO: 8952 - RNA, 20 nt, synthetic construct
  source 1..20: mol_type = other RNA
tgtaatcccagcactttggg

SEQ ID NO: 8953 - RNA, 20 nt, synthetic construct
  source 1..20: mol_type = other RNA
gcctgtaatcccagcacttt

SEQ ID NO: 8954 - RNA, 20 nt, synthetic construct
  source 1..20: mol_type = other RNA
cgcctgtaatcccagcactt

SEQ ID NO: 8955 - RNA, 20 nt, synthetic construct
  source 1..20: mol_type = other RNA
caggcgtgagccaccacgct

SEQ ID NO: 8956 - RNA, 20 nt, synthetic construct
  source 1..20: mol_type = other RNA
tggttattggccgagcgtgg

SEQ ID NO: 8957 - RNA, 20 nt, synthetic construct
  source 1..20: mol_type = other RNA
ttgtggttattggccgagcg

SEQ ID NO: 8958 - RNA, 20 nt, synthetic construct
  source 1..20: mol_type = other RNA
actttaaagattgtggttat

SEQ ID NO: 8959 - RNA, 20 nt, synthetic construct
  source 1..20: mol_type = other RNA
acaatgaactttaaagattg

SEQ ID NO: 8960 - RNA, 20 nt, synthetic construct
  source 1..20: mol_type = other RNA
tctattaactttaaaaacaa

SEQ ID NO: 8961 - RNA, 20 nt, synthetic construct
  source 1..20: mol_type = other RNA
taactttaaaaacaaaggaa

SEQ ID NO: 8962 - RNA, 20 nt, synthetic construct
  source 1..20: mol_type = other RNA
tttaaaaacaaaggaatggt

SEQ ID NO: 8963 - RNA, 20 nt, synthetic construct
  source 1..20: mol_type = other RNA
ttaaaaacaaaggaatggtt

SEQ ID NO: 8964 - RNA, 20 nt, synthetic construct
  source 1..20: mol_type = other RNA
ttgggcagatttgtctatta

SEQ ID NO: 8965 - RNA, 20 nt, synthetic construct
  source 1..20: mol_type = other RNA
tatggaatcagaccagcagc

SEQ ID NO: 8966 - RNA, 20 nt, synthetic construct
  source 1..20: mol_type = other RNA
gaatcagaccagcagcagga

SEQ ID NO: 8967 - RNA, 20 nt, synthetic construct
  source 1..20: mol_type = other RNA
aatcagaccagcagcaggaa

SEQ ID NO: 8968 - RNA, 20 nt, synthetic construct
  source 1..20: mol_type = other RNA
agcagcaggaagggctcaat

SEQ ID NO: 8969 - RNA, 20 nt, synthetic construct
  source 1..20: mol_type = other RNA
aattgagcccttcctgctgc

SEQ ID NO: 8970 - RNA, 20 nt, synthetic construct
  source 1..20: mol_type = other RNA
ggaaagtgctgagaatccca

SEQ ID NO: 8971 - RNA, 20 nt, synthetic construct
  source 1..20: mol_type = other RNA
gagaatcccacggcttcgat

SEQ ID NO: 8972 - RNA, 20 nt, synthetic construct
  source 1..20: mol_type = other RNA
cacggcttcgatcggttgta

SEQ ID NO: 8973 - RNA, 20 nt, synthetic construct
  source 1..20: mol_type = other RNA
acggcttcgatcggttgtat

SEQ ID NO: 8974 - RNA, 20 nt, synthetic construct
  source 1..20: mol_type = other RNA
atacaaccgatcgaagccgt

SEQ ID NO: 8975 - RNA, 20 nt, synthetic construct
  source 1..20: mol_type = other RNA
catacaaccgatcgaagccg

SEQ ID NO: 8976 - RNA, 20 nt, synthetic construct
  source 1..20: mol_type = other RNA
agtcgtacatggattctaac

SEQ ID NO: 8977 - RNA, 20 nt, synthetic construct
  source 1..20: mol_type = other RNA
tctggctaaaaagtcgtaca

SEQ ID NO: 8978 - RNA, 20 nt, synthetic construct
  source 1..20: mol_type = other RNA
attttttctgggagaagctc

SEQ ID NO: 8979 - RNA, 20 nt, synthetic construct
  source 1..20: mol_type = other RNA
tgaaaagtctgattttttct

SEQ ID NO: 8980 - RNA, 20 nt, synthetic construct
  source 1..20: mol_type = other RNA
gtgaaaagtctgattttttc

SEQ ID NO: 8981 - RNA, 20 nt, synthetic construct
  source 1..20: mol_type = other RNA
gacttttcacaaatatattt

SEQ ID NO: 8982 - RNA, 20 nt, synthetic construct
  source 1..20: mol_type = other RNA
gttaaaagtatactaaccca

SEQ ID NO: 8983 - RNA, 20 nt, synthetic construct
  source 1..20: mol_type = other RNA
aaaaaaaaaattcttacctt

SEQ ID NO: 8984 - RNA, 20 nt, synthetic construct
  source 1..20: mol_type = other RNA
aaaaaaaaaaattcttacct

SEQ ID NO: 8985 - RNA, 20 nt, synthetic construct
  source 1..20: mol_type = other RNA
attttgaagagtttatactc

SEQ ID NO: 8986 - RNA, 20 nt, synthetic construct
  source 1..20: mol_type = other RNA
gagtttatactcaggcatag

SEQ ID NO: 8987 - RNA, 20 nt, synthetic construct
  source 1..20: mol_type = other RNA
atcccttctttctgttttct

SEQ ID NO: 8988 - RNA, 20 nt, synthetic construct
  source 1..20: mol_type = other RNA
ccttctttctgttttcttgg

SEQ ID NO: 8989 - RNA, 20 nt, synthetic construct
  source 1..20: mol_type = other RNA
cttctttctgttttcttggt

SEQ ID NO: 8990 - RNA, 20 nt, synthetic construct
  source 1..20: mol_type = other RNA
caccaagaaaacagaaagaa

SEQ ID NO: 8991 - RNA, 20 nt, synthetic construct
  source 1..20: mol_type = other RNA
ccaccaagaaaacagaaaga

SEQ ID NO: 8992 - RNA, 20 nt, synthetic construct
  source 1..20: mol_type = other RNA
ttctgttttcttggtgggaa

SEQ ID NO: 8993 - RNA, 20 nt, synthetic construct
  source 1..20: mol_type = other RNA
tgggaaaggcagaagcagag

SEQ ID NO: 8994 - RNA, 20 nt, synthetic construct
  source 1..20: mol_type = other RNA
aaggcagaagcagagaggtc

SEQ ID NO: 8995 - RNA, 20 nt, synthetic construct
  source 1..20: mol_type = other RNA
aagcagagaggtcaggagaa

SEQ ID NO: 8996 - RNA, 20 nt, synthetic construct
  source 1..20: mol_type = other RNA
agaggtcaggagaaaggaga

SEQ ID NO: 8997 - RNA, 20 nt, synthetic construct
  source 1..20: mol_type = other RNA
gaggtcaggagaaaggagat

SEQ ID NO: 8998 - RNA, 20 nt, synthetic construct
  source 1..20: mol_type = other RNA
aggtcaggagaaaggagatg

SEQ ID NO: 8999 - RNA, 20 nt, synthetic construct
  source 1..20: mol_type = other RNA
caggagaaaggagatgggga

SEQ ID NO: 9000 - RNA, 20 nt, synthetic construct
  source 1..20: mol_type = other RNA
gatggggacggataacagca

SEQ ID NO: 9001 - RNA, 20 nt, synthetic construct
  source 1..20: mol_type = other RNA
ggggacggataacagcatgg

SEQ ID NO: 9002 - RNA, 20 nt, synthetic construct
  source 1..20: mol_type = other RNA
gggacggataacagcatggt

SEQ ID NO: 9003 - RNA, 20 nt, synthetic construct
  source 1..20: mol_type = other RNA
acagcatggtgggcagtgcc

SEQ ID NO: 9004 - RNA, 20 nt, synthetic construct
  source 1..20: mol_type = other RNA
gtgggcagtgccaggcatgc

SEQ ID NO: 9005 - RNA, 20 nt, synthetic construct
  source 1..20: mol_type = other RNA
tgggcagtgccaggcatgct

SEQ ID NO: 9006 - RNA, 20 nt, synthetic construct
  source 1..20: mol_type = other RNA
agaaacacacccagcatgcc

SEQ ID NO: 9007 - RNA, 20 nt, synthetic construct
  source 1..20: mol_type = other RNA
gtgtttctgtttgaatgtcc

SEQ ID NO: 9008 - RNA, 20 nt, synthetic construct
  source 1..20: mol_type = other RNA
gaatgtccaggctgtgacaa

SEQ ID NO: 9009 - RNA, 20 nt, synthetic construct
  source 1..20: mol_type = other RNA
aatgtccaggctgtgacaaa

SEQ ID NO: 9010 - RNA, 20 nt, synthetic construct
  source 1..20: mol_type = other RNA
ggctgtgacaaagggaagta

SEQ ID NO: 9011 - RNA, 20 nt, synthetic construct
  source 1..20: mol_type = other RNA
tacttccctttgtcacagcc

SEQ ID NO: 9012 - RNA, 20 nt, synthetic construct
  source 1..20: mol_type = other RNA
gggaagtaaggaatgcatgt

SEQ ID NO: 9013 - RNA, 20 nt, synthetic construct
  source 1..20: mol_type = other RNA
aagtaaggaatgcatgttgg

SEQ ID NO: 9014 - RNA, 20 nt, synthetic construct
  source 1..20: mol_type = other RNA
agtaaggaatgcatgttgga

SEQ ID NO: 9015 - RNA, 20 nt, synthetic construct
  source 1..20: mol_type = other RNA
catgagggcaaatgagaaat

SEQ ID NO: 9016 - RNA, 20 nt, synthetic construct
  source 1..20: mol_type = other RNA
acatgagggcaaatgagaaa

SEQ ID NO: 9017 - RNA, 20 nt, synthetic construct
  source 1..20: mol_type = other RNA
ctcatttgccctcatgtcta

SEQ ID NO: 9018 - RNA, 20 nt, synthetic construct
  source 1..20: mol_type = other RNA
ccctcatgtctagggcccag

SEQ ID NO: 9019 - RNA, 20 nt, synthetic construct
  source 1..20: mol_type = other RNA
cctctgggccctagacatga

SEQ ID NO: 9020 - RNA, 20 nt, synthetic construct
  source 1..20: mol_type = other RNA
tcctctgggccctagacatg

SEQ ID NO: 9021 - RNA, 20 nt, synthetic construct
  source 1..20: mol_type = other RNA
gcccagaggaccagtcactt

SEQ ID NO: 9022 - RNA, 20 nt, synthetic construct
  source 1..20: mol_type = other RNA
tcctaagtgactggtcctct

SEQ ID NO: 9023 - RNA, 20 nt, synthetic construct
  source 1..20: mol_type = other RNA
gtcctaagtgactggtcctc

SEQ ID NO: 9024 - RNA, 20 nt, synthetic construct
  source 1..20: mol_type = other RNA
cttcagctgtcctaagtgac

SEQ ID NO: 9025 - RNA, 20 nt, synthetic construct
  source 1..20: mol_type = other RNA
caagcaactgttgacatttc

SEQ ID NO: 9026 - RNA, 20 nt, synthetic construct
  source 1..20: mol_type = other RNA
cagaaatgtcaacagttgct

SEQ ID NO: 9027 - RNA, 20 nt, synthetic construct
  source 1..20: mol_type = other RNA
gtgagggagaagaggagaca

SEQ ID NO: 9028 - RNA, 20 nt, synthetic construct
  source 1..20: mol_type = other RNA
tcattttggtgagggagaag

SEQ ID NO: 9029 - RNA, 20 nt, synthetic construct
  source 1..20: mol_type = other RNA
ctcaccaaaatgatattagc

SEQ ID NO: 9030 - RNA, 20 nt, synthetic construct
  source 1..20: mol_type = other RNA
tcaccaaaatgatattagct

SEQ ID NO: 9031 - RNA, 20 nt, synthetic construct
  source 1..20: mol_type = other RNA
agctaatatcattttggtga

SEQ ID NO: 9032 - RNA, 20 nt, synthetic construct
  source 1..20: mol_type = other RNA
cagctaatatcattttggtg

SEQ ID NO: 9033 - RNA, 20 nt, synthetic construct
  source 1..20: mol_type = other RNA
agtcccagctaatatcattt

SEQ ID NO: 9034 - RNA, 20 nt, synthetic construct
  source 1..20: mol_type = other RNA
tgcattgtggataggaggtg

SEQ ID NO: 9035 - RNA, 20 nt, synthetic construct
  source 1..20: mol_type = other RNA
gggaatgcattgtggatagg

SEQ ID NO: 9036 - RNA, 20 nt, synthetic construct
  source 1..20: mol_type = other RNA
acagggaatgcattgtggat

SEQ ID NO: 9037 - RNA, 20 nt, synthetic construct
  source 1..20: mol_type = other RNA
gcagacagcacaagcctcaa

SEQ ID NO: 9038 - RNA, 20 nt, synthetic construct
  source 1..20: mol_type = other RNA
tctggggaatatggcctttg

SEQ ID NO: 9039 - RNA, 20 nt, synthetic construct
  source 1..20: mol_type = other RNA
tgattacattctggggaata

SEQ ID NO: 9040 - RNA, 20 nt, synthetic construct
  source 1..20: mol_type = other RNA
agtaggatgattacattctg

SEQ ID NO: 9041 - RNA, 20 nt, synthetic construct
  source 1..20: mol_type = other RNA
aagtaggatgattacattct

SEQ ID NO: 9042 - RNA, 20 nt, synthetic construct
  source 1..20: mol_type = other RNA
aaagtaggatgattacattc

SEQ ID NO: 9043 - RNA, 20 nt, synthetic construct
  source 1..20: mol_type = other RNA
atcttcggtatttcaaaagt

SEQ ID NO: 9044 - RNA, 20 nt, synthetic construct
  source 1..20: mol_type = other RNA
tcattgtactattatatctt

SEQ ID NO: 9045 - RNA, 20 nt, synthetic construct
  source 1..20: mol_type = other RNA
aaatattcttaccccgatga

SEQ ID NO: 9046 - RNA, 20 nt, synthetic construct
  source 1..20: mol_type = other RNA
attcttaccccgatgaaggc

SEQ ID NO: 9047 - RNA, 20 nt, synthetic construct
  source 1..20: mol_type = other RNA
atgaaggctggctccagttg

SEQ ID NO: 9048 - RNA, 20 nt, synthetic construct
  source 1..20: mol_type = other RNA
aactggagccagccttcatc

SEQ ID NO: 9049 - RNA, 20 nt, synthetic construct
  source 1..20: mol_type = other RNA
caactggagccagccttcat

SEQ ID NO: 9050 - RNA, 20 nt, synthetic construct
  source 1..20: mol_type = other RNA
ttgacttgctaagccacaac

SEQ ID NO: 9051 - RNA, 20 nt, synthetic construct
  source 1..20: mol_type = other RNA
gaattttaggatgttgttac

SEQ ID NO: 9052 - RNA, 20 nt, synthetic construct
  source 1..20: mol_type = other RNA
acaacatcctaaaattccaa

SEQ ID NO: 9053 - RNA, 20 nt, synthetic construct
  source 1..20: mol_type = other RNA
agaataacctttggaatttt

SEQ ID NO: 9054 - RNA, 20 nt, synthetic construct
  source 1..20: mol_type = other RNA
ggatggggaagaataacctt

SEQ ID NO: 9055 - RNA, 20 nt, synthetic construct
  source 1..20: mol_type = other RNA
tggctttttaactgtggatg

SEQ ID NO: 9056 - RNA, 20 nt, synthetic construct
  source 1..20: mol_type = other RNA
atggctttttaactgtggat

SEQ ID NO: 9057 - RNA, 20 nt, synthetic construct
  source 1..20: mol_type = other RNA
gatggctttttaactgtgga

SEQ ID NO: 9058 - RNA, 20 nt, synthetic construct
  source 1..20: mol_type = other RNA
aggagatggctttttaactg

SEQ ID NO: 9059 - RNA, 20 nt, synthetic construct
  source 1..20: mol_type = other RNA
tgacactgttctgtaggaga

SEQ ID NO: 9060 - RNA, 20 nt, synthetic construct
  source 1..20: mol_type = other RNA
cagatatgacactgttctgt

SEQ ID NO: 9061 - RNA, 20 nt, synthetic construct
  source 1..20: mol_type = other RNA
tgtgacatgtccaagattaa

SEQ ID NO: 9062 - RNA, 20 nt, synthetic construct
  source 1..20: mol_type = other RNA
gaaggctcttcctttaatct

SEQ ID NO: 9063 - RNA, 20 nt, synthetic construct
  source 1..20: mol_type = other RNA
cttgcttttagtaatttgtc

SEQ ID NO: 9064 - RNA, 20 nt, synthetic construct
  source 1..20: mol_type = other RNA
acaaattactaaaagcaaga

SEQ ID NO: 9065 - RNA, 20 nt, synthetic construct
  source 1..20: mol_type = other RNA
aaagccatcttcatgcttca

SEQ ID NO: 9066 - RNA, 20 nt, synthetic construct
  source 1..20: mol_type = other RNA
aagccatcttcatgcttcat

SEQ ID NO: 9067 - RNA, 20 nt, synthetic construct
  source 1..20: mol_type = other RNA
tctcccatgaagcatgaaga

SEQ ID NO: 9068 - RNA, 20 nt, synthetic construct
  source 1..20: mol_type = other RNA
aatgtgtgatttttaaacag

SEQ ID NO: 9069 - RNA, 20 nt, synthetic construct
  source 1..20: mol_type = other RNA
atctgatacttgatacgaag

SEQ ID NO: 9070 - RNA, 20 nt, synthetic construct
  source 1..20: mol_type = other RNA
tttttttgcatttcagcacg

SEQ ID NO: 9071 - RNA, 20 nt, synthetic construct
  source 1..20: mol_type = other RNA
gcacgaggcaaacaaacaaa

SEQ ID NO: 9072 - RNA, 20 nt, synthetic construct
  source 1..20: mol_type = other RNA
aagacgcgtttgaaacttcg

SEQ ID NO: 9073 - RNA, 20 nt, synthetic construct
  source 1..20: mol_type = other RNA
tagtaacataaactgaagtt

SEQ ID NO: 9074 - RNA, 20 nt, synthetic construct
  source 1..20: mol_type = other RNA
tggtaattcaatatcaaaga

SEQ ID NO: 9075 - RNA, 20 nt, synthetic construct
  source 1..20: mol_type = other RNA
tttttttcagcgagatactt

SEQ ID NO: 9076 - RNA, 20 nt, synthetic construct
  source 1..20: mol_type = other RNA
cttgtttattaattgcaagg

SEQ ID NO: 9077 - RNA, 20 nt, synthetic construct
  source 1..20: mol_type = other RNA
acttgtttattaattgcaag

SEQ ID NO: 9078 - RNA, 20 nt, synthetic construct
  source 1..20: mol_type = other RNA
aacttgtttattaattgcaa

SEQ ID NO: 9079 - RNA, 20 nt, synthetic construct
  source 1..20: mol_type = other RNA
caacttgtttattaattgca

SEQ ID NO: 9080 - RNA, 20 nt, synthetic construct
  source 1..20: mol_type = other RNA
aatgtgaagattcttagctt

SEQ ID NO: 9081 - RNA, 20 nt, synthetic construct
  source 1..20: mol_type = other RNA
attccaaatctttccattcc

SEQ ID NO: 9082 - RNA, 20 nt, synthetic construct
  source 1..20: mol_type = other RNA
cttccaggaatggaaagatt

SEQ ID NO: 9083 - RNA, 20 nt, synthetic construct
  source 1..20: mol_type = other RNA
ttccattcctggaagagctt

SEQ ID NO: 9084 - RNA, 20 nt, synthetic construct
  source 1..20: mol_type = other RNA
taccaaagctcttccaggaa

SEQ ID NO: 9085 - RNA, 20 nt, synthetic construct
  source 1..20: mol_type = other RNA
ctaaataccaaagctcttcc

SEQ ID NO: 9086 - RNA, 20 nt, synthetic construct
  source 1..20: mol_type = other RNA
tttggtatttagatgttaat

SEQ ID NO: 9087 - RNA, 20 nt, synthetic construct
  source 1..20: mol_type = other RNA
aagaaaaaaaaaaaaaaggc

SEQ ID NO: 9088 - RNA, 20 nt, synthetic construct
  source 1..20: mol_type = other RNA
tttttttttttttctttttt

SEQ ID NO: 9089 - RNA, 20 nt, synthetic construct
  source 1..20: mol_type = other RNA
aaaaaagaaaaaaaaaaaaa

SEQ ID NO: 9090 - RNA, 20 nt, synthetic construct
  source 1..20: mol_type = other RNA
tctttttttggccaatcttc

SEQ ID NO: 9091 - RNA, 20 nt, synthetic construct
  source 1..20: mol_type = other RNA
agactctttagcctgaagat

SEQ ID NO: 9092 - RNA, 20 nt, synthetic construct
  source 1..20: mol_type = other RNA
catcctatgacctcagtttt

SEQ ID NO: 9093 - RNA, 20 nt, synthetic construct
  source 1..20: mol_type = other RNA
ctaaaactgaggtcatagga

SEQ ID NO: 9094 - RNA, 20 nt, synthetic construct
  source 1..20: mol_type = other RNA
aatcctaaaactgaggtcat

SEQ ID NO: 9095 - RNA, 20 nt, synthetic construct
  source 1..20: mol_type = other RNA
agaaagaaatcctaaaactg

SEQ ID NO: 9096 - RNA, 20 nt, synthetic construct
  source 1..20: mol_type = other RNA
cttgcaaaatttagttattt

SEQ ID NO: 9097 - RNA, 20 nt, synthetic construct
  source 1..20: mol_type = other RNA
caaaatttagttattttggt

SEQ ID NO: 9098 - RNA, 20 nt, synthetic construct
  source 1..20: mol_type = other RNA
aagaaaataagaatgaattc

SEQ ID NO: 9099 - RNA, 20 nt, synthetic construct
  source 1..20: mol_type = other RNA
tcttattttctttctccttc

SEQ ID NO: 9100 - RNA, 20 nt, synthetic construct
  source 1..20: mol_type = other RNA
taaagggagaaagtaccaga

SEQ ID NO: 9101 - RNA, 20 nt, synthetic construct
  source 1..20: mol_type = other RNA
gagaaacagaagggggtaaa

SEQ ID NO: 9102 - RNA, 20 nt, synthetic construct
  source 1..20: mol_type = other RNA
agagaaacagaagggggtaa

SEQ ID NO: 9103 - RNA, 20 nt, synthetic construct
  source 1..20: mol_type = other RNA
gaagggagagaaacagaagg

SEQ ID NO: 9104 - RNA, 20 nt, synthetic construct
  source 1..20: mol_type = other RNA
agaagggagagaaacagaag

SEQ ID NO: 9105 - RNA, 20 nt, synthetic construct
  source 1..20: mol_type = other RNA
aagaagggagagaaacagaa

SEQ ID NO: 9106 - RNA, 20 nt, synthetic construct
  source 1..20: mol_type = other RNA
gaagaagggagagaaacaga

SEQ ID NO: 9107 - RNA, 20 nt, synthetic construct
  source 1..20: mol_type = other RNA
aatacaagataggtgaagaa

SEQ ID NO: 9108 - RNA, 20 nt, synthetic construct
  source 1..20: mol_type = other RNA
taatacaagataggtgaaga

SEQ ID NO: 9109 - RNA, 20 nt, synthetic construct
  source 1..20: mol_type = other RNA
ttcagagaataatacaagat

SEQ ID NO: 9110 - RNA, 20 nt, synthetic construct
  source 1..20: mol_type = other RNA
tgaattaagaatttaaagtc

SEQ ID NO: 9111 - RNA, 20 nt, synthetic construct
  source 1..20: mol_type = other RNA
ttaagaatttaaagtccggt

SEQ ID NO: 9112 - RNA, 20 nt, synthetic construct
  source 1..20: mol_type = other RNA
agaatttaaagtccggttgg

SEQ ID NO: 9113 - RNA, 20 nt, synthetic construct
  source 1..20: mol_type = other RNA
ttaaagtccggttggtggac

SEQ ID NO: 9114 - RNA, 20 nt, synthetic construct
  source 1..20: mol_type = other RNA
ctgtagtccagtccaccaac

SEQ ID NO: 9115 - RNA, 20 nt, synthetic construct
  source 1..20: mol_type = other RNA
actacagtctctatgatgtt

SEQ ID NO: 9116 - RNA, 20 nt, synthetic construct
  source 1..20: mol_type = other RNA
cagtctctatgatgtttggt

SEQ ID NO: 9117 - RNA, 20 nt, synthetic construct
  source 1..20: mol_type = other RNA
agtctctatgatgtttggta

SEQ ID NO: 9118 - RNA, 20 nt, synthetic construct
  source 1..20: mol_type = other RNA
gaattagcaaatgaaaatac

SEQ ID NO: 9119 - RNA, 20 nt, synthetic construct
  source 1..20: mol_type = other RNA
cctagttaaatttgaatttc

SEQ ID NO: 9120 - RNA, 20 nt, synthetic construct
  source 1..20: mol_type = other RNA
cctgaaattcaaatttaact

SEQ ID NO: 9121 - RNA, 20 nt, synthetic construct
  source 1..20: mol_type = other RNA
atgtgtctcatgcaatattt

SEQ ID NO: 9122 - RNA, 20 nt, synthetic construct
  source 1..20: mol_type = other RNA
aatgtgtctcatgcaatatt

SEQ ID NO: 9123 - RNA, 20 nt, synthetic construct
  source 1..20: mol_type = other RNA
aattattttcaagtattgca

SEQ ID NO: 9124 - RNA, 20 nt, synthetic construct
  source 1..20: mol_type = other RNA
attattttcaagtattgcat

SEQ ID NO: 9125 - RNA, 20 nt, synthetic construct
  source 1..20: mol_type = other RNA
atctgaaattcaaatttaac

SEQ ID NO: 9126 - RNA, 20 nt, synthetic construct
  source 1..20: mol_type = other RNA
tctgaaattcaaatttaact

SEQ ID NO: 9127 - RNA, 20 nt, synthetic construct
  source 1..20: mol_type = other RNA
tgggcgtcttatattttatc

SEQ ID NO: 9128 - RNA, 20 nt, synthetic construct
  source 1..20: mol_type = other RNA
tttatctggcaacactactt

SEQ ID NO: 9129 - RNA, 20 nt, synthetic construct
  source 1..20: mol_type = other RNA
atctggcaacactactttgg

SEQ ID NO: 9130 - RNA, 20 nt, synthetic construct
  source 1..20: mol_type = other RNA
acactactttggaggttcaa

SEQ ID NO: 9131 - RNA, 20 nt, synthetic construct
  source 1..20: mol_type = other RNA
tactttggaggttcaatgga

SEQ ID NO: 9132 - RNA, 20 nt, synthetic construct
  source 1..20: mol_type = other RNA
actttggaggttcaatggaa

SEQ ID NO: 9133 - RNA, 20 nt, synthetic construct
  source 1..20: mol_type = other RNA
agggattttaaaaaaaacaa

SEQ ID NO: 9134 - RNA, 20 nt, synthetic construct
  source 1..20: mol_type = other RNA
aggcatccatttacaactcc

SEQ ID NO: 9135 - RNA, 20 nt, synthetic construct
  source 1..20: mol_type = other RNA
cttcttccaggagttgtaaa

SEQ ID NO: 9136 - RNA, 20 nt, synthetic construct
  source 1..20: mol_type = other RNA
gtggaaatttctcttcttcc

SEQ ID NO: 9137 - RNA, 20 nt, synthetic construct
  source 1..20: mol_type = other RNA
agcgttcaagaggataggag

SEQ ID NO: 9138 - RNA, 20 nt, synthetic construct
  source 1..20: mol_type = other RNA
caaaaagcgttcaagaggat

SEQ ID NO: 9139 - RNA, 20 nt, synthetic construct
  source 1..20: mol_type = other RNA
ctagacaaaaagcgttcaag

SEQ ID NO: 9140 - RNA, 20 nt, synthetic construct
  source 1..20: mol_type = other RNA
gtcaaaaataaactaaaatg

SEQ ID NO: 9141 - RNA, 20 nt, synthetic construct
  source 1..20: mol_type = other RNA
agcttttagtacaacttact

SEQ ID NO: 9142 - RNA, 20 nt, synthetic construct
  source 1..20: mol_type = other RNA
gagcttttagtacaacttac

SEQ ID NO: 9143 - RNA, 20 nt, synthetic construct
  source 1..20: mol_type = other RNA
taaggatgtgacatgctctg

SEQ ID NO: 9144 - RNA, 20 nt, synthetic construct
  source 1..20: mol_type = other RNA
atattaaagaagtccatccc

SEQ ID NO: 9145 - RNA, 20 nt, synthetic construct
  source 1..20: mol_type = other RNA
ggatggacttctttaatata

SEQ ID NO: 9146 - RNA, 20 nt, synthetic construct
  source 1..20: mol_type = other RNA
agaagtccatcccaggtttc

SEQ ID NO: 9147 - RNA, 20 nt, synthetic construct
  source 1..20: mol_type = other RNA
cccaggtttcaggtctcact

SEQ ID NO: 9148 - RNA, 20 nt, synthetic construct
  source 1..20: mol_type = other RNA
gtgagacctgaaacctggga

SEQ ID NO: 9149 - RNA, 20 nt, synthetic construct
  source 1..20: mol_type = other RNA
ccgagtgagacctgaaacct

SEQ ID NO: 9150 - RNA, 20 nt, synthetic construct
  source 1..20: mol_type = other RNA
accgagtgagacctgaaacc

SEQ ID NO: 9151 - RNA, 20 nt, synthetic construct
  source 1..20: mol_type = other RNA
ttcaggtctcactcggtgtc

SEQ ID NO: 9152 - RNA, 20 nt, synthetic construct
  source 1..20: mol_type = other RNA
gtctcactcggtgtcaggcc

SEQ ID NO: 9153 - RNA, 20 nt, synthetic construct
  source 1..20: mol_type = other RNA
caggccagagcttgcaaaat

SEQ ID NO: 9154 - RNA, 20 nt, synthetic construct
  source 1..20: mol_type = other RNA
caattttgcaagctctggcc

SEQ ID NO: 9155 - RNA, 20 nt, synthetic construct
  source 1..20: mol_type = other RNA
gggaccaattttgcaagctc

SEQ ID NO: 9156 - RNA, 20 nt, synthetic construct
  source 1..20: mol_type = other RNA
aattggtcccccaggcaaca

SEQ ID NO: 9157 - RNA, 20 nt, synthetic construct
  source 1..20: mol_type = other RNA
attggtcccccaggcaacat

SEQ ID NO: 9158 - RNA, 20 nt, synthetic construct
  source 1..20: mol_type = other RNA
ccccaggcaacatgggacct

SEQ ID NO: 9159 - RNA, 20 nt, synthetic construct
  source 1..20: mol_type = other RNA
caaggtcccatgttgcctgg

SEQ ID NO: 9160 - RNA, 20 nt, synthetic construct
  source 1..20: mol_type = other RNA
ccaaggtcccatgttgcctg

SEQ ID NO: 9161 - RNA, 20 nt, synthetic construct
  source 1..20: mol_type = other RNA
gccaaggtcccatgttgcct

SEQ ID NO: 9162 - RNA, 20 nt, synthetic construct
  source 1..20: mol_type = other RNA
cgccaaggtcccatgttgcc

SEQ ID NO: 9163 - RNA, 20 nt, synthetic construct
  source 1..20: mol_type = other RNA
attgttctgttactgcgcca

SEQ ID NO: 9164 - RNA, 20 nt, synthetic construct
  source 1..20: mol_type = other RNA
ttgaaggaaaaaattaaaac

SEQ ID NO: 9165 - RNA, 20 nt, synthetic construct
  source 1..20: mol_type = other RNA
atttggtgttcagattttga

SEQ ID NO: 9166 - RNA, 20 nt, synthetic construct
  source 1..20: mol_type = other RNA
accaaatttagtacttttga

SEQ ID NO: 9167 - RNA, 20 nt, synthetic construct
  source 1..20: mol_type = other RNA
gccttcaaaagtactaaatt

SEQ ID NO: 9168 - RNA, 20 nt, synthetic construct
  source 1..20: mol_type = other RNA
tctctcctcagtgctcactt

SEQ ID NO: 9169 - RNA, 20 nt, synthetic construct
  source 1..20: mol_type = other RNA
ctctcctcagtgctcacttt

SEQ ID NO: 9170 - RNA, 20 nt, synthetic construct
  source 1..20: mol_type = other RNA
tctcctcagtgctcactttg

SEQ ID NO: 9171 - RNA, 20 nt, synthetic construct
  source 1..20: mol_type = other RNA
ttgccccaaagtgagcactg

SEQ ID NO: 9172 - RNA, 20 nt, synthetic construct
  source 1..20: mol_type = other RNA
acattcatgtgaattctatt

SEQ ID NO: 9173 - RNA, 20 nt, synthetic construct
  source 1..20: mol_type = other RNA
aacattcatgtgaattctat

SEQ ID NO: 9174 - RNA, 20 nt, synthetic construct
  source 1..20: mol_type = other RNA
gtaataaaatgatcactttt

SEQ ID NO: 9175 - RNA, 20 nt, synthetic construct
  source 1..20: mol_type = other RNA
taataaaatgatcacttttt

SEQ ID NO: 9176 - RNA, 20 nt, synthetic construct
  source 1..20: mol_type = other RNA
cactttttgggcattttgaa

SEQ ID NO: 9177 - RNA, 20 nt, synthetic construct
  source 1..20: mol_type = other RNA
actttttgggcattttgaaa

SEQ ID NO: 9178 - RNA, 20 nt, synthetic construct
  source 1..20: mol_type = other RNA
attacattaattattaattc

SEQ ID NO: 9179 - RNA, 20 nt, synthetic construct
  source 1..20: mol_type = other RNA
ctgaacatctaaagaaaccc

SEQ ID NO: 9180 - RNA, 20 nt, synthetic construct
  source 1..20: mol_type = other RNA
aacatctaaagaaacccagg

SEQ ID NO: 9181 - RNA, 20 nt, synthetic construct
  source 1..20: mol_type = other RNA
acatctaaagaaacccagga

SEQ ID NO: 9182 - RNA, 20 nt, synthetic construct
  source 1..20: mol_type = other RNA
gaattatgtgtcgccctcct

SEQ ID NO: 9183 - RNA, 20 nt, synthetic construct
  source 1..20: mol_type = other RNA
ggaattatgtgtcgccctcc

SEQ ID NO: 9184 - RNA, 20 nt, synthetic construct
  source 1..20: mol_type = other RNA
taaataagagaacggcattt

SEQ ID NO: 9185 - RNA, 20 nt, synthetic construct
  source 1..20: mol_type = other RNA
tgtgtctctaaataagagaa

SEQ ID NO: 9186 - RNA, 20 nt, synthetic construct
  source 1..20: mol_type = other RNA
cacattgatattcagtattt

SEQ ID NO: 9187 - RNA, 20 nt, synthetic construct
  source 1..20: mol_type = other RNA
ttgaagtttaatagctgaaa

SEQ ID NO: 9188 - RNA, 20 nt, synthetic construct
  source 1..20: mol_type = other RNA
aagtttaatagctgaaatgg

SEQ ID NO: 9189 - RNA, 20 nt, synthetic construct
  source 1..20: mol_type = other RNA
tgtactttaaattcttaaac

SEQ ID NO: 9190 - RNA, 20 nt, synthetic construct
  source 1..20: mol_type = other RNA
ttcaaagaataatacaagat

SEQ ID NO: 9191 - RNA, 20 nt, synthetic construct
  source 1..20: mol_type = other RNA
taatacaagataggtgaaga

SEQ ID NO: 9192 - RNA, 20 nt, synthetic construct
  source 1..20: mol_type = other RNA
gaagaaggaagagaaacaga

SEQ ID NO: 9193 - RNA, 20 nt, synthetic construct
  source 1..20: mol_type = other RNA
aagaaggaagagaaacagaa

SEQ ID NO: 9194 - RNA, 20 nt, synthetic construct
  source 1..20: mol_type = other RNA
agaaggaagagaaacagaag

SEQ ID NO: 9195 - RNA, 20 nt, synthetic construct
  source 1..20: mol_type = other RNA
gaaggaagagaaacagaagg

SEQ ID NO: 9196 - RNA, 20 nt, synthetic construct
  source 1..20: mol_type = other RNA
agagaaacagaagggggtaa

SEQ ID NO: 9197 - RNA, 20 nt, synthetic construct
  source 1..20: mol_type = other RNA
gagaaacagaagggggtaaa

SEQ ID NO: 9198 - RNA, 20 nt, synthetic construct
  source 1..20: mol_type = other RNA
taaagggagaaagtaccaga

SEQ ID NO: 9199 - RNA, 20 nt, synthetic construct
  source 1..20: mol_type = other RNA
gattattttgtttctccttc

SEQ ID NO: 9200 - RNA, 20 nt, synthetic construct
  source 1..20: mol_type = other RNA
tgatgatggaaggaagccca

SEQ ID NO: 9201 - RNA, 20 nt, synthetic construct
  source 1..20: mol_type = other RNA
atagtaataatgatgatgga

SEQ ID NO: 9202 - RNA, 20 nt, synthetic construct
  source 1..20: mol_type = other RNA
tgtaatagtaataatgatga

SEQ ID NO: 9203 - RNA, 20 nt, synthetic construct
  source 1..20: mol_type = other RNA
ttgcactatctcattttatg

SEQ ID NO: 9204 - RNA, 20 nt, synthetic construct
  source 1..20: mol_type = other RNA
tatgaggcatatttaagaac

SEQ ID NO: 9205 - RNA, 20 nt, synthetic construct
  source 1..20: mol_type = other RNA
gtattcgatgtgccattgtc

SEQ ID NO: 9206 - RNA, 20 nt, synthetic construct
  source 1..20: mol_type = other RNA
gtgccattgtctggactctc

SEQ ID NO: 9207 - RNA, 20 nt, synthetic construct
  source 1..20: mol_type = other RNA
gagccagagagtccagacaa

SEQ ID NO: 9208 - RNA, 20 nt, synthetic construct
  source 1..20: mol_type = other RNA
gcatcacctttctcttaaaa

SEQ ID NO: 9209 - RNA, 20 nt, synthetic construct
  source 1..20: mol_type = other RNA
ctgcttcctttttaagagaa

SEQ ID NO: 9210 - RNA, 20 nt, synthetic construct
  source 1..20: mol_type = other RNA
agactgtaagactcatatgt

SEQ ID NO: 9211 - RNA, 20 nt, synthetic construct
  source 1..20: mol_type = other RNA
aaagattgttaataggagca

SEQ ID NO: 9212 - RNA, 20 nt, synthetic construct
  source 1..20: mol_type = other RNA
cattttgaaagattgttaat

SEQ ID NO: 9213 - RNA, 20 nt, synthetic construct
  source 1..20: mol_type = other RNA
aatctttcaaaatgtgtagc

SEQ ID NO: 9214 - RNA, 20 nt, synthetic construct
  source 1..20: mol_type = other RNA
ctttcaaaatgtgtagcagg

SEQ ID NO: 9215 - RNA, 20 nt, synthetic construct
  source 1..20: mol_type = other RNA
agaaattcactaaaaaactg

SEQ ID NO: 9216 - RNA, 20 nt, synthetic construct
  source 1..20: mol_type = other RNA
aagaaattcactaaaaaact

SEQ ID NO: 9217 - RNA, 20 nt, synthetic construct
  source 1..20: mol_type = other RNA
aaagaaattcactaaaaaac

SEQ ID NO: 9218 - RNA, 20 nt, synthetic construct
  source 1..20: mol_type = other RNA
atgagcacacattggacagt

SEQ ID NO: 9219 - RNA, 20 nt, synthetic construct
  source 1..20: mol_type = other RNA
gagggaggatgagcacacat

SEQ ID NO: 9220 - RNA, 20 nt, synthetic construct
  source 1..20: mol_type = other RNA
cagagggcagaaggggaggg

SEQ ID NO: 9221 - RNA, 20 nt, synthetic construct
  source 1..20: mol_type = other RNA
gggcagagggcagaagggga

SEQ ID NO: 9222 - RNA, 20 nt, synthetic construct
  source 1..20: mol_type = other RNA
ggggcagagggcagaagggg

SEQ ID NO: 9223 - RNA, 20 nt, synthetic construct
  source 1..20: mol_type = other RNA
gtgggggcagagggcagaag

SEQ ID NO: 9224 - RNA, 20 nt, synthetic construct
  source 1..20: mol_type = other RNA
ggtgggggcagagggcagaa

SEQ ID NO: 9225 - RNA, 20 nt, synthetic construct
  source 1..20: mol_type = other RNA
gggtgggggcagagggcaga

SEQ ID NO: 9226 - RNA, 20 nt, synthetic construct
  source 1..20: mol_type = other RNA
gagcagggggtgggggcaga

SEQ ID NO: 9227 - RNA, 20 nt, synthetic construct
  source 1..20: mol_type = other RNA
ggagcagggggtgggggcag

SEQ ID NO: 9228 - RNA, 20 nt, synthetic construct
  source 1..20: mol_type = other RNA
atctggggagcagggggtgg

SEQ ID NO: 9229 - RNA, 20 nt, synthetic construct
  source 1..20: mol_type = other RNA
catctggggagcagggggtg

SEQ ID NO: 9230 - RNA, 20 nt, synthetic construct
  source 1..20: mol_type = other RNA
tcatctggggagcagggggt

SEQ ID NO: 9231 - RNA, 20 nt, synthetic construct
  source 1..20: mol_type = other RNA
ttcatctggggagcaggggg

SEQ ID NO: 9232 - RNA, 20 nt, synthetic construct
  source 1..20: mol_type = other RNA
agtttcatctggggagcagg

SEQ ID NO: 9233 - RNA, 20 nt, synthetic construct
  source 1..20: mol_type = other RNA
gagtttcatctggggagcag

SEQ ID NO: 9234 - RNA, 20 nt, synthetic construct
  source 1..20: mol_type = other RNA
ggagtttcatctggggagca

SEQ ID NO: 9235 - RNA, 20 nt, synthetic construct
  source 1..20: mol_type = other RNA
tggagtttcatctggggagc

SEQ ID NO: 9236 - RNA, 20 nt, synthetic construct
  source 1..20: mol_type = other RNA
tcgctctggagtttcatctg

SEQ ID NO: 9237 - RNA, 20 nt, synthetic construct
  source 1..20: mol_type = other RNA
ttcgctctggagtttcatct

SEQ ID NO: 9238 - RNA, 20 nt, synthetic construct
  source 1..20: mol_type = other RNA
cttcgctctggagtttcatc

SEQ ID NO: 9239 - RNA, 20 nt, synthetic construct
  source 1..20: mol_type = other RNA
agagcgaagtctttcttact

SEQ ID NO: 9240 - RNA, 20 nt, synthetic construct
  source 1..20: mol_type = other RNA
aagtaagaaagacttcgctc

SEQ ID NO: 9241 - RNA, 20 nt, synthetic construct
  source 1..20: mol_type = other RNA
acttggattattgtgtccag

SEQ ID NO: 9242 - RNA, 20 nt, synthetic construct
  source 1..20: mol_type = other RNA
gactctcagcttgtatcctc

SEQ ID NO: 9243 - RNA, 20 nt, synthetic construct
  source 1..20: mol_type = other RNA
ttgatatttcttgttctttc

SEQ ID NO: 9244 - RNA, 20 nt, synthetic construct
  source 1..20: mol_type = other RNA
acatgatctcatgtttaact

SEQ ID NO: 9245 - RNA, 20 nt, synthetic construct
  source 1..20: mol_type = other RNA
catgagatcatgtttaaaac

SEQ ID NO: 9246 - RNA, 20 nt, synthetic construct
  source 1..20: mol_type = other RNA
agagattgagagcaatgaat

SEQ ID NO: 9247 - RNA, 20 nt, synthetic construct
  source 1..20: mol_type = other RNA
tctgtaaatattcctgccag

SEQ ID NO: 9248 - RNA, 20 nt, synthetic construct
  source 1..20: mol_type = other RNA
tacagaagaaaagacaatca

SEQ ID NO: 9249 - RNA, 20 nt, synthetic construct
  source 1..20: mol_type = other RNA
acagaagaaaagacaatcac

SEQ ID NO: 9250 - RNA, 20 nt, synthetic construct
  source 1..20: mol_type = other RNA
aggcatttctagtgggcagt

SEQ ID NO: 9251 - RNA, 20 nt, synthetic construct
  source 1..20: mol_type = other RNA
caggcatttctagtgggcag

SEQ ID NO: 9252 - RNA, 20 nt, synthetic construct
  source 1..20: mol_type = other RNA
ctcatgcaggcatttctagt

SEQ ID NO: 9253 - RNA, 20 nt, synthetic construct
  source 1..20: mol_type = other RNA
actcatgcaggcatttctag

SEQ ID NO: 9254 - RNA, 20 nt, synthetic construct
  source 1..20: mol_type = other RNA
ggaatatgtttcactcatgc

SEQ ID NO: 9255 - RNA, 20 nt, synthetic construct
  source 1..20: mol_type = other RNA
agtgaaacatattcctcctg

SEQ ID NO: 9256 - RNA, 20 nt, synthetic construct
  source 1..20: mol_type = other RNA
gtgaaacatattcctcctga

SEQ ID NO: 9257 - RNA, 20 nt, synthetic construct
  source 1..20: mol_type = other RNA
gagatcttgcatccctcagg

SEQ ID NO: 9258 - RNA, 20 nt, synthetic construct
  source 1..20: mol_type = other RNA
ggtgagatcttgcatccctc

SEQ ID NO: 9259 - RNA, 20 nt, synthetic construct
  source 1..20: mol_type = other RNA
atgcaagatctcaccttatt

SEQ ID NO: 9260 - RNA, 20 nt, synthetic construct
  source 1..20: mol_type = other RNA
gatctcaccttatttggaaa

SEQ ID NO: 9261 - RNA, 20 nt, synthetic construct
  source 1..20: mol_type = other RNA
cttatttggaaatggaaatt

SEQ ID NO: 9262 - RNA, 20 nt, synthetic construct
  source 1..20: mol_type = other RNA
caaatttccatttccaaata

SEQ ID NO: 9263 - RNA, 20 nt, synthetic construct
  source 1..20: mol_type = other RNA
ttggttggttccactttgcc

SEQ ID NO: 9264 - RNA, 20 nt, synthetic construct
  source 1..20: mol_type = other RNA
tattcaagcacctggcaaag

SEQ ID NO: 9265 - RNA, 20 nt, synthetic construct
  source 1..20: mol_type = other RNA
ggtgcttgaatagcagaaag

SEQ ID NO: 9266 - RNA, 20 nt, synthetic construct
  source 1..20: mol_type = other RNA
ctttctgctattcaagcacc

SEQ ID NO: 9267 - RNA, 20 nt, synthetic construct
  source 1..20: mol_type = other RNA
gcttgaatagcagaaagtgg

SEQ ID NO: 9268 - RNA, 20 nt, synthetic construct
  source 1..20: mol_type = other RNA
agcagaaagtggtggaagcc

SEQ ID NO: 9269 - RNA, 20 nt, synthetic construct
  source 1..20: mol_type = other RNA
gaagccaggtcatctcctga

SEQ ID NO: 9270 - RNA, 20 nt, synthetic construct
  source 1..20: mol_type = other RNA
ccaggtcatctcctgaagga

SEQ ID NO: 9271 - RNA, 20 nt, synthetic construct
  source 1..20: mol_type = other RNA
caggtcatctcctgaaggac

SEQ ID NO: 9272 - RNA, 20 nt, synthetic construct
  source 1..20: mol_type = other RNA
ccgtccttcaggagatgacc

SEQ ID NO: 9273 - RNA, 20 nt, synthetic construct
  source 1..20: mol_type = other RNA
ttgtttttatcccgtccttc

SEQ ID NO: 9274 - RNA, 20 nt, synthetic construct
  source 1..20: mol_type = other RNA
cagacagtatttaaaatcag

SEQ ID NO: 9275 - RNA, 20 nt, synthetic construct
  source 1..20: mol_type = other RNA
atgtaaagcagctgtacaag

SEQ ID NO: 9276 - RNA, 20 nt, synthetic construct
  source 1..20: mol_type = other RNA
tgtaaagcagctgtacaagt

SEQ ID NO: 9277 - RNA, 20 nt, synthetic construct
  source 1..20: mol_type = other RNA
tgtacaagtgggccttcata

SEQ ID NO: 9278 - RNA, 20 nt, synthetic construct
  source 1..20: mol_type = other RNA
caagtgggccttcataaggc

SEQ ID NO: 9279 - RNA, 20 nt, synthetic construct
  source 1..20: mol_type = other RNA
aagtgggccttcataaggca

SEQ ID NO: 9280 - RNA, 20 nt, synthetic construct
  source 1..20: mol_type = other RNA
gggccttcataaggcaggga

SEQ ID NO: 9281 - RNA, 20 nt, synthetic construct
  source 1..20: mol_type = other RNA
ggccttcataaggcagggaa

SEQ ID NO: 9282 - RNA, 20 nt, synthetic construct
  source 1..20: mol_type = other RNA
aacccttccctgccttatga

SEQ ID NO: 9283 - RNA, 20 nt, synthetic construct
  source 1..20: mol_type = other RNA
aagggttaaaaaatgtacaa

SEQ ID NO: 9284 - RNA, 20 nt, synthetic construct
  source 1..20: mol_type = other RNA
aaatgtcaaaccacagacta

SEQ ID NO: 9285 - RNA, 20 nt, synthetic construct
  source 1..20: mol_type = other RNA
aatgtcaaaccacagactat

SEQ ID NO: 9286 - RNA, 20 nt, synthetic construct
  source 1..20: mol_type = other RNA
gactatgggctcctttatca

SEQ ID NO: 9287 - RNA, 20 nt, synthetic construct
  source 1..20: mol_type = other RNA
ctcctttatcatggagccgc

SEQ ID NO: 9288 - RNA, 20 nt, synthetic construct
  source 1..20: mol_type = other RNA
aacctgcggctccatgataa

SEQ ID NO: 9289 - RNA, 20 nt, synthetic construct
  source 1..20: mol_type = other RNA
ctaaatagaaaggaaacctg

SEQ ID NO: 9290 - RNA, 20 nt, synthetic construct
  source 1..20: mol_type = other RNA
gacatagactctaaatagaa

SEQ ID NO: 9291 - RNA, 20 nt, synthetic construct
  source 1..20: mol_type = other RNA
aaacagtcttatcaatctgt

SEQ ID NO: 9292 - RNA, 20 nt, synthetic construct
  source 1..20: mol_type = other RNA
taaacagtcttatcaatctg

SEQ ID NO: 9293 - RNA, 20 nt, synthetic construct
  source 1..20: mol_type = other RNA
gtttaaagaataatcttacc

SEQ ID NO: 9294 - RNA, 20 nt, synthetic construct
  source 1..20: mol_type = other RNA
ctgtgttgaagaaataatcc

SEQ ID NO: 9295 - RNA, 20 nt, synthetic construct
  source 1..20: mol_type = other RNA
gctgtgttgaagaaataatc

SEQ ID NO: 9296 - RNA, 20 nt, synthetic construct
  source 1..20: mol_type = other RNA
tatttcttcaacacagctgt

SEQ ID NO: 9297 - RNA, 20 nt, synthetic construct
  source 1..20: mol_type = other RNA
tgctttcaggagagtagatc

SEQ ID NO: 9298 - RNA, 20 nt, synthetic construct
  source 1..20: mol_type = other RNA
atttttttttctttgctttc

SEQ ID NO: 9299 - RNA, 20 nt, synthetic construct
  source 1..20: mol_type = other RNA
gaaaaaaaaattaagcctga

SEQ ID NO: 9300 - RNA, 20 nt, synthetic construct
  source 1..20: mol_type = other RNA
ggtcatcaatctattccatc

SEQ ID NO: 9301 - RNA, 20 nt, synthetic construct
  source 1..20: mol_type = other RNA
gaccacacagaagacatgca

SEQ ID NO: 9302 - RNA, 20 nt, synthetic construct
  source 1..20: mol_type = other RNA
aaccttgcatgtcttctgtg

SEQ ID NO: 9303 - RNA, 20 nt, synthetic construct
  source 1..20: mol_type = other RNA
tttgttgggggggactaatt

SEQ ID NO: 9304 - RNA, 20 nt, synthetic construct
  source 1..20: mol_type = other RNA
gctgaatttttttgttgggg

SEQ ID NO: 9305 - RNA, 20 nt, synthetic construct
  source 1..20: mol_type = other RNA
cgctgaatttttttgttggg

SEQ ID NO: 9306 - RNA, 20 nt, synthetic construct
  source 1..20: mol_type = other RNA
tcgctgaatttttttgttgg

SEQ ID NO: 9307 - RNA, 20 nt, synthetic construct
  source 1..20: mol_type = other RNA
ctcgctgaatttttttgttg

SEQ ID NO: 9308 - RNA, 20 nt, synthetic construct
  source 1..20: mol_type = other RNA
actcgctgaatttttttgtt

SEQ ID NO: 9309 - RNA, 20 nt, synthetic construct
  source 1..20: mol_type = other RNA
aactcgctgaatttttttgt

SEQ ID NO: 9310 - RNA, 20 nt, synthetic construct
  source 1..20: mol_type = other RNA
attcagcgagttacaggttg

SEQ ID NO: 9311 - RNA, 20 nt, synthetic construct
  source 1..20: mol_type = other RNA
ttcagcgagttacaggttga

SEQ ID NO: 9312 - RNA, 20 nt, synthetic construct
  source 1..20: mol_type = other RNA
tcagcgagttacaggttgag

SEQ ID NO: 9313 - RNA, 20 nt, synthetic construct
  source 1..20: mol_type = other RNA
gtggccagtgacaaggagct

SEQ ID NO: 9314 - RNA, 20 nt, synthetic construct
  source 1..20: mol_type = other RNA
ggagctgggagcttgccctg

SEQ ID NO: 9315 - RNA, 20 nt, synthetic construct
  source 1..20: mol_type = other RNA
gagctgggagcttgccctga

SEQ ID NO: 9316 - RNA, 20 nt, synthetic construct
  source 1..20: mol_type = other RNA
gagcttgccctgagggcagc

SEQ ID NO: 9317 - RNA, 20 nt, synthetic construct
  source 1..20: mol_type = other RNA
cttgccctgagggcagcagg

SEQ ID NO: 9318 - RNA, 20 nt, synthetic construct
  source 1..20: mol_type = other RNA
ctgagggcagcaggaggcca

SEQ ID NO: 9319 - RNA, 20 nt, synthetic construct
  source 1..20: mol_type = other RNA
tgagggcagcaggaggccat

SEQ ID NO: 9320 - RNA, 20 nt, synthetic construct
  source 1..20: mol_type = other RNA
atggcctcctgctgccctca

SEQ ID NO: 9321 - RNA, 20 nt, synthetic construct
  source 1..20: mol_type = other RNA
catggcctcctgctgccctc

SEQ ID NO: 9322 - RNA, 20 nt, synthetic construct
  source 1..20: mol_type = other RNA
aggccatgggcaagcagaga

SEQ ID NO: 9323 - RNA, 20 nt, synthetic construct
  source 1..20: mol_type = other RNA
ggccatgggcaagcagagaa

SEQ ID NO: 9324 - RNA, 20 nt, synthetic construct
  source 1..20: mol_type = other RNA
tgggcaagcagagaagggac

SEQ ID NO: 9325 - RNA, 20 nt, synthetic construct
  source 1..20: mol_type = other RNA
gggcaagcagagaagggaca

SEQ ID NO: 9326 - RNA, 20 nt, synthetic construct
  source 1..20: mol_type = other RNA
gtcccttctctgcttgccca

SEQ ID NO: 9327 - RNA, 20 nt, synthetic construct
  source 1..20: mol_type = other RNA
aagcagagaagggacagggt

SEQ ID NO: 9328 - RNA, 20 nt, synthetic construct
  source 1..20: mol_type = other RNA
gactttcagaaacagtcctc

SEQ ID NO: 9329 - RNA, 20 nt, synthetic construct
  source 1..20: mol_type = other RNA
acagtcctctggttgctaaa

SEQ ID NO: 9330 - RNA, 20 nt, synthetic construct
  source 1..20: mol_type = other RNA
cagtcctctggttgctaaat

SEQ ID NO: 9331 - RNA, 20 nt, synthetic construct
  source 1..20: mol_type = other RNA
ctggttgctaaatgggagaa

SEQ ID NO: 9332 - RNA, 20 nt, synthetic construct
  source 1..20: mol_type = other RNA
ttctcccatttagcaaccag

SEQ ID NO: 9333 - RNA, 20 nt, synthetic construct
  source 1..20: mol_type = other RNA
ggagaaaggagtgacagtag

SEQ ID NO: 9334 - RNA, 20 nt, synthetic construct
  source 1..20: mol_type = other RNA
aaaggagtgacagtagaggc

SEQ ID NO: 9335 - RNA, 20 nt, synthetic construct
  source 1..20: mol_type = other RNA
gtgacagtagaggcaggaga

SEQ ID NO: 9336 - RNA, 20 nt, synthetic construct
  source 1..20: mol_type = other RNA
cagtagaggcaggagaaggc

SEQ ID NO: 9337 - RNA, 20 nt, synthetic construct
  source 1..20: mol_type = other RNA
caggagaaggcaggatcaga

SEQ ID NO: 9338 - RNA, 20 nt, synthetic construct
  source 1..20: mol_type = other RNA
aggagaaggcaggatcagac

SEQ ID NO: 9339 - RNA, 20 nt, synthetic construct
  source 1..20: mol_type = other RNA
ggagaaggcaggatcagacg

SEQ ID NO: 9340 - RNA, 20 nt, synthetic construct
  source 1..20: mol_type = other RNA
gagaaggcaggatcagacgg

SEQ ID NO: 9341 - RNA, 20 nt, synthetic construct
  source 1..20: mol_type = other RNA
gcaggatcagacgggggtgc

SEQ ID NO: 9342 - RNA, 20 nt, synthetic construct
  source 1..20: mol_type = other RNA
caggatcagacgggggtgct

SEQ ID NO: 9343 - RNA, 20 nt, synthetic construct
  source 1..20: mol_type = other RNA
atcagacgggggtgctggga

SEQ ID NO: 9344 - RNA, 20 nt, synthetic construct
  source 1..20: mol_type = other RNA
tcagacgggggtgctgggaa

SEQ ID NO: 9345 - RNA, 20 nt, synthetic construct
  source 1..20: mol_type = other RNA
cagacgggggtgctgggaag

SEQ ID NO: 9346 - RNA, 20 nt, synthetic construct
  source 1..20: mol_type = other RNA
cgggggtgctgggaaggggc

SEQ ID NO: 9347 - RNA, 20 nt, synthetic construct
  source 1..20: mol_type = other RNA
gggcaggtagaagagacatc

SEQ ID NO: 9348 - RNA, 20 nt, synthetic construct
  source 1..20: mol_type = other RNA
caggtagaagagacatcagg

SEQ ID NO: 9349 - RNA, 20 nt, synthetic construct
  source 1..20: mol_type = other RNA
catcaggaggccaaacagat

SEQ ID NO: 9350 - RNA, 20 nt, synthetic construct
  source 1..20: mol_type = other RNA
atcataaagtcctatctgtt

SEQ ID NO: 9351 - RNA, 20 nt, synthetic construct
  source 1..20: mol_type = other RNA
aggactttatgatgcaccgt

SEQ ID NO: 9352 - RNA, 20 nt, synthetic construct
  source 1..20: mol_type = other RNA
tttgggtactggtataccta

SEQ ID NO: 9353 - RNA, 20 nt, synthetic construct
  source 1..20: mol_type = other RNA
gtataccagtacccaaacac

SEQ ID NO: 9354 - RNA, 20 nt, synthetic construct
  source 1..20: mol_type = other RNA
taccagtacccaaacacagg

SEQ ID NO: 9355 - RNA, 20 nt, synthetic construct
  source 1..20: mol_type = other RNA
ggccacctgtgtttgggtac

SEQ ID NO: 9356 - RNA, 20 nt, synthetic construct
  source 1..20: mol_type = other RNA
gctcttggccacctgtgttt

SEQ ID NO: 9357 - RNA, 20 nt, synthetic construct
  source 1..20: mol_type = other RNA
tgctcttggccacctgtgtt

SEQ ID NO: 9358 - RNA, 20 nt, synthetic construct
  source 1..20: mol_type = other RNA
ggcgtctatccctctgctct

SEQ ID NO: 9359 - RNA, 20 nt, synthetic construct
  source 1..20: mol_type = other RNA
atgtctgtgaggaggaggct

SEQ ID NO: 9360 - RNA, 20 nt, synthetic construct
  source 1..20: mol_type = other RNA
gatgtctgtgaggaggaggc

SEQ ID NO: 9361 - RNA, 20 nt, synthetic construct
  source 1..20: mol_type = other RNA
cctggatgtctgtgaggagg

SEQ ID NO: 9362 - RNA, 20 nt, synthetic construct
  source 1..20: mol_type = other RNA
atgcctggatgtctgtgagg

SEQ ID NO: 9363 - RNA, 20 nt, synthetic construct
  source 1..20: mol_type = other RNA
tgcatgcctggatgtctgtg

SEQ ID NO: 9364 - RNA, 20 nt, synthetic construct
  source 1..20: mol_type = other RNA
cgtggagggctctgcatgcc

SEQ ID NO: 9365 - RNA, 20 nt, synthetic construct
  source 1..20: mol_type = other RNA
cctccacgtgccaaacacac

SEQ ID NO: 9366 - RNA, 20 nt, synthetic construct
  source 1..20: mol_type = other RNA
ctccacgtgccaaacacaca

SEQ ID NO: 9367 - RNA, 20 nt, synthetic construct
  source 1..20: mol_type = other RNA
ctgtgtgtttggcacgtgga

SEQ ID NO: 9368 - RNA, 20 nt, synthetic construct
  source 1..20: mol_type = other RNA
cctgtgtgtttggcacgtgg

SEQ ID NO: 9369 - RNA, 20 nt, synthetic construct
  source 1..20: mol_type = other RNA
gtgccaaacacacagggccg

SEQ ID NO: 9370 - RNA, 20 nt, synthetic construct
  source 1..20: mol_type = other RNA
ggccctgtgtgtttggcacg

SEQ ID NO: 9371 - RNA, 20 nt, synthetic construct
  source 1..20: mol_type = other RNA
aaacacacagggccgaggaa

SEQ ID NO: 9372 - RNA, 20 nt, synthetic construct
  source 1..20: mol_type = other RNA
attcctcggccctgtgtgtt

SEQ ID NO: 9373 - RNA, 20 nt, synthetic construct
  source 1..20: mol_type = other RNA
tctgctgcacttccattcct

SEQ ID NO: 9374 - RNA, 20 nt, synthetic construct
  source 1..20: mol_type = other RNA
gtgcagcagagccgatacgc

SEQ ID NO: 9375 - RNA, 20 nt, synthetic construct
  source 1..20: mol_type = other RNA
cagatctgctgcctgcgtat

SEQ ID NO: 9376 - RNA, 20 nt, synthetic construct
  source 1..20: mol_type = other RNA
gcagcagatctgcaataacc

SEQ ID NO: 9377 - RNA, 20 nt, synthetic construct
  source 1..20: mol_type = other RNA
ggacacacagtcccaccaga

SEQ ID NO: 9378 - RNA, 20 nt, synthetic construct
  source 1..20: mol_type = other RNA
tctggtgggactgtgtgtcc

SEQ ID NO: 9379 - RNA, 20 nt, synthetic construct
  source 1..20: mol_type = other RNA
ccaccagaaggagagagcag

SEQ ID NO: 9380 - RNA, 20 nt, synthetic construct
  source 1..20: mol_type = other RNA
cactgctctctccttctggt

SEQ ID NO: 9381 - RNA, 20 nt, synthetic construct
  source 1..20: mol_type = other RNA
ccactgctctctccttctgg

SEQ ID NO: 9382 - RNA, 20 nt, synthetic construct
  source 1..20: mol_type = other RNA
attccactgctctctccttc

SEQ ID NO: 9383 - RNA, 20 nt, synthetic construct
  source 1..20: mol_type = other RNA
gagagagcagtggaatgatc

SEQ ID NO: 9384 - RNA, 20 nt, synthetic construct
  source 1..20: mol_type = other RNA
agagagcagtggaatgatca

SEQ ID NO: 9385 - RNA, 20 nt, synthetic construct
  source 1..20: mol_type = other RNA
tcactgcagcctcgatctct

SEQ ID NO: 9386 - RNA, 20 nt, synthetic construct
  source 1..20: mol_type = other RNA
cgcttgagtccaagagatcg

SEQ ID NO: 9387 - RNA, 20 nt, synthetic construct
  source 1..20: mol_type = other RNA
actagggaggctggagtgag

SEQ ID NO: 9388 - RNA, 20 nt, synthetic construct
  source 1..20: mol_type = other RNA
actccagcctccctagtagc

SEQ ID NO: 9389 - RNA, 20 nt, synthetic construct
  source 1..20: mol_type = other RNA
ctccagcctccctagtagct

SEQ ID NO: 9390 - RNA, 20 nt, synthetic construct
  source 1..20: mol_type = other RNA
gtcccagctactagggaggc

SEQ ID NO: 9391 - RNA, 20 nt, synthetic construct
  source 1..20: mol_type = other RNA
tccctagtagctgggaccac

SEQ ID NO: 9392 - RNA, 20 nt, synthetic construct
  source 1..20: mol_type = other RNA
tgtggtcccagctactaggg

SEQ ID NO: 9393 - RNA, 20 nt, synthetic construct
  source 1..20: mol_type = other RNA
gcctgtggtcccagctacta

SEQ ID NO: 9394 - RNA, 20 nt, synthetic construct
  source 1..20: mol_type = other RNA
tgcctgtggtcccagctact

SEQ ID NO: 9395 - RNA, 20 nt, synthetic construct
  source 1..20: mol_type = other RNA
caggcacacgccatgatacc

SEQ ID NO: 9396 - RNA, 20 nt, synthetic construct
  source 1..20: mol_type = other RNA
ggtatcatggcgtgtgcctg

SEQ ID NO: 9397 - RNA, 20 nt, synthetic construct
  source 1..20: mol_type = other RNA
taaaacttaaccaggtatca

SEQ ID NO: 9398 - RNA, 20 nt, synthetic construct
  source 1..20: mol_type = other RNA
ttaaaaattaaaacttaacc

SEQ ID NO: 9399 - RNA, 20 nt, synthetic construct
  source 1..20: mol_type = other RNA
ttttaaacttcttgtagaga

SEQ ID NO: 9400 - RNA, 20 nt, synthetic construct
  source 1..20: mol_type = other RNA
tttaaacttcttgtagagat

SEQ ID NO: 9401 - RNA, 20 nt, synthetic construct
  source 1..20: mol_type = other RNA
ttaaacttcttgtagagatg

SEQ ID NO: 9402 - RNA, 20 nt, synthetic construct
  source 1..20: mol_type = other RNA
taaacttcttgtagagatgg

SEQ ID NO: 9403 - RNA, 20 nt, synthetic construct
  source 1..20: mol_type = other RNA
tctcagtgcattgaccagtc

SEQ ID NO: 9404 - RNA, 20 nt, synthetic construct
  source 1..20: mol_type = other RNA
ccagtctggtctcgaactcc

SEQ ID NO: 9405 - RNA, 20 nt, synthetic construct
  source 1..20: mol_type = other RNA
cagtctggtctcgaactcct

SEQ ID NO: 9406 - RNA, 20 nt, synthetic construct
  source 1..20: mol_type = other RNA
ccaggagttcgagaccagac

SEQ ID NO: 9407 - RNA, 20 nt, synthetic construct
  source 1..20: mol_type = other RNA
tgggaggatcgcttgagccc

SEQ ID NO: 9408 - RNA, 20 nt, synthetic construct
  source 1..20: mol_type = other RNA
ctcaagcgatcctcccacct

SEQ ID NO: 9409 - RNA, 20 nt, synthetic construct
  source 1..20: mol_type = other RNA
ctttgggaggccaaggtggg

SEQ ID NO: 9410 - RNA, 20 nt, synthetic construct
  source 1..20: mol_type = other RNA
accttggcctcccaaagtgc

SEQ ID NO: 9411 - RNA, 20 nt, synthetic construct
  source 1..20: mol_type = other RNA
ccttggcctcccaaagtgct

SEQ ID NO: 9412 - RNA, 20 nt, synthetic construct
  source 1..20: mol_type = other RNA
gcactttgggaggccaaggt

SEQ ID NO: 9413 - RNA, 20 nt, synthetic construct
  source 1..20: mol_type = other RNA
agcactttgggaggccaagg

SEQ ID NO: 9414 - RNA, 20 nt, synthetic construct
  source 1..20: mol_type = other RNA
cccagcactttgggaggcca

SEQ ID NO: 9415 - RNA, 20 nt, synthetic construct
  source 1..20: mol_type = other RNA
tcccaaagtgctgggattac

SEQ ID NO: 9416 - RNA, 20 nt, synthetic construct
  source 1..20: mol_type = other RNA
tgtaatcccagcactttggg

SEQ ID NO: 9417 - RNA, 20 nt, synthetic construct
  source 1..20: mol_type = other RNA
tcctgtaatcccagcacttt

SEQ ID NO: 9418 - RNA, 20 nt, synthetic construct
  source 1..20: mol_type = other RNA
ctcctgtaatcccagcactt

SEQ ID NO: 9419 - RNA, 20 nt, synthetic construct
  source 1..20: mol_type = other RNA
caggagtgagttactgtgcc

SEQ ID NO: 9420 - RNA, 20 nt, synthetic construct
  source 1..20: mol_type = other RNA
aataagaatagttgttggcc

SEQ ID NO: 9421 - RNA, 20 nt, synthetic construct
  source 1..20: mol_type = other RNA
gaataagaatagttgttggc

SEQ ID NO: 9422 - RNA, 20 nt, synthetic construct
  source 1..20: mol_type = other RNA
atgggaataagaatagttgt

SEQ ID NO: 9423 - RNA, 20 nt, synthetic construct
  source 1..20: mol_type = other RNA
tcttattcccattttacaga

SEQ ID NO: 9424 - RNA, 20 nt, synthetic construct
  source 1..20: mol_type = other RNA
ttttacagatggacaaactg

SEQ ID NO: 9425 - RNA, 20 nt, synthetic construct
  source 1..20: mol_type = other RNA
agtttgtccatctgtaaaat

SEQ ID NO: 9426 - RNA, 20 nt, synthetic construct
  source 1..20: mol_type = other RNA
cagtttgtccatctgtaaaa

SEQ ID NO: 9427 - RNA, 20 nt, synthetic construct
  source 1..20: mol_type = other RNA
agatggacaaactgaggctc

SEQ ID NO: 9428 - RNA, 20 nt, synthetic construct
  source 1..20: mol_type = other RNA
tggacaaactgaggctcagg

SEQ ID NO: 9429 - RNA, 20 nt, synthetic construct
  source 1..20: mol_type = other RNA
gtgggctacaggcaagtgac

SEQ ID NO: 9430 - RNA, 20 nt, synthetic construct
  source 1..20: mol_type = other RNA
tgcctgtagcccacagttag

SEQ ID NO: 9431 - RNA, 20 nt, synthetic construct
  source 1..20: mol_type = other RNA
taccactaactgtgggctac

SEQ ID NO: 9432 - RNA, 20 nt, synthetic construct
  source 1..20: mol_type = other RNA
cccacagttagtggtagcac

SEQ ID NO: 9433 - RNA, 20 nt, synthetic construct
  source 1..20: mol_type = other RNA
ccacagttagtggtagcact

SEQ ID NO: 9434 - RNA, 20 nt, synthetic construct
  source 1..20: mol_type = other RNA
ccagtgctaccactaactgt

SEQ ID NO: 9435 - RNA, 20 nt, synthetic construct
  source 1..20: mol_type = other RNA
cccagtgctaccactaactg

SEQ ID NO: 9436 - RNA, 20 nt, synthetic construct
  source 1..20: mol_type = other RNA
gtagcactgggattccaact

SEQ ID NO: 9437 - RNA, 20 nt, synthetic construct
  source 1..20: mol_type = other RNA
tagcactgggattccaactt

SEQ ID NO: 9438 - RNA, 20 nt, synthetic construct
  source 1..20: mol_type = other RNA
gacatgaaggggacccaagt

SEQ ID NO: 9439 - RNA, 20 nt, synthetic construct
  source 1..20: mol_type = other RNA
cccttcatgtcgcctgtatt

SEQ ID NO: 9440 - RNA, 20 nt, synthetic construct
  source 1..20: mol_type = other RNA
caaatacaggcgacatgaag

SEQ ID NO: 9441 - RNA, 20 nt, synthetic construct
  source 1..20: mol_type = other RNA
ccaaatacaggcgacatgaa

SEQ ID NO: 9442 - RNA, 20 nt, synthetic construct
  source 1..20: mol_type = other RNA
accaaatacaggcgacatga

SEQ ID NO: 9443 - RNA, 20 nt, synthetic construct
  source 1..20: mol_type = other RNA
ctgtatttggtgtcccattt

SEQ ID NO: 9444 - RNA, 20 nt, synthetic construct
  source 1..20: mol_type = other RNA
ctaaatgggacaccaaatac

SEQ ID NO: 9445 - RNA, 20 nt, synthetic construct
  source 1..20: mol_type = other RNA
tcccatttaggcgtccatgc

SEQ ID NO: 9446 - RNA, 20 nt, synthetic construct
  source 1..20: mol_type = other RNA
acctgcatggacgcctaaat

SEQ ID NO: 9447 - RNA, 20 nt, synthetic construct
  source 1..20: mol_type = other RNA
aacctgcatggacgcctaaa

SEQ ID NO: 9448 - RNA, 20 nt, synthetic construct
  source 1..20: mol_type = other RNA
cagacacgccaaaacctgca

SEQ ID NO: 9449 - RNA, 20 nt, synthetic construct
  source 1..20: mol_type = other RNA
ccccaagtaagtgtccccca

SEQ ID NO: 9450 - RNA, 20 nt, synthetic construct
  source 1..20: mol_type = other RNA
ccatgggggacacttacttg

SEQ ID NO: 9451 - RNA, 20 nt, synthetic construct
  source 1..20: mol_type = other RNA
tccatgggggacacttactt

SEQ ID NO: 9452 - RNA, 20 nt, synthetic construct
  source 1..20: mol_type = other RNA
atccatgggggacacttact

SEQ ID NO: 9453 - RNA, 20 nt, synthetic construct
  source 1..20: mol_type = other RNA
ggctgggtgggcatccatgg

SEQ ID NO: 9454 - RNA, 20 nt, synthetic construct
  source 1..20: mol_type = other RNA
cggctgggtgggcatccatg

SEQ ID NO: 9455 - RNA, 20 nt, synthetic construct
  source 1..20: mol_type = other RNA
acggctgggtgggcatccat

SEQ ID NO: 9456 - RNA, 20 nt, synthetic construct
  source 1..20: mol_type = other RNA
cacggctgggtgggcatcca

SEQ ID NO: 9457 - RNA, 20 nt, synthetic construct
  source 1..20: mol_type = other RNA
acaggaggacacggctgggt

SEQ ID NO: 9458 - RNA, 20 nt, synthetic construct
  source 1..20: mol_type = other RNA
gacaggaggacacggctggg

SEQ ID NO: 9459 - RNA, 20 nt, synthetic construct
  source 1..20: mol_type = other RNA
gccgtgtcctcctgtctctg

SEQ ID NO: 9460 - RNA, 20 nt, synthetic construct
  source 1..20: mol_type = other RNA
agagacaggaggacacggct

SEQ ID NO: 9461 - RNA, 20 nt, synthetic construct
  source 1..20: mol_type = other RNA
cagagacaggaggacacggc

SEQ ID NO: 9462 - RNA, 20 nt, synthetic construct
  source 1..20: mol_type = other RNA
acctcagagacaggaggaca

SEQ ID NO: 9463 - RNA, 20 nt, synthetic construct
  source 1..20: mol_type = other RNA
cctgtctctgaggtttctcc

SEQ ID NO: 9464 - RNA, 20 nt, synthetic construct
  source 1..20: mol_type = other RNA
ggagaaacctcagagacagg

SEQ ID NO: 9465 - RNA, 20 nt, synthetic construct
  source 1..20: mol_type = other RNA
cctggagaaacctcagagac

SEQ ID NO: 9466 - RNA, 20 nt, synthetic construct
  source 1..20: mol_type = other RNA
ttctccaggaatcgagctcc

SEQ ID NO: 9467 - RNA, 20 nt, synthetic construct
  source 1..20: mol_type = other RNA
caggaatcgagctcctggcc

SEQ ID NO: 9468 - RNA, 20 nt, synthetic construct
  source 1..20: mol_type = other RNA
caggccaggagctcgattcc

SEQ ID NO: 9469 - RNA, 20 nt, synthetic construct
  source 1..20: mol_type = other RNA
acactcagacaagccaggcc

SEQ ID NO: 9470 - RNA, 20 nt, synthetic construct
  source 1..20: mol_type = other RNA
ggcttgtctgagtgtgtctg

SEQ ID NO: 9471 - RNA, 20 nt, synthetic construct
  source 1..20: mol_type = other RNA
gcttgtctgagtgtgtctgt

SEQ ID NO: 9472 - RNA, 20 nt, synthetic construct
  source 1..20: mol_type = other RNA
cagacacactcagacaagcc

SEQ ID NO: 9473 - RNA, 20 nt, synthetic construct
  source 1..20: mol_type = other RNA
gtagcatgcccctgcccgtc

SEQ ID NO: 9474 - RNA, 20 nt, synthetic construct
  source 1..20: mol_type = other RNA
tagcatgcccctgcccgtct

SEQ ID NO: 9475 - RNA, 20 nt, synthetic construct
  source 1..20: mol_type = other RNA
gacgggcaggggcatgctac

SEQ ID NO: 9476 - RNA, 20 nt, synthetic construct
  source 1..20: mol_type = other RNA
agagggacccagacgggcag

SEQ ID NO: 9477 - RNA, 20 nt, synthetic construct
  source 1..20: mol_type = other RNA
cagagggacccagacgggca

SEQ ID NO: 9478 - RNA, 20 nt, synthetic construct
  source 1..20: mol_type = other RNA
gcagagggacccagacgggc

SEQ ID NO: 9479 - RNA, 20 nt, synthetic construct
  source 1..20: mol_type = other RNA
acacgcagagggacccagac

SEQ ID NO: 9480 - RNA, 20 nt, synthetic construct
  source 1..20: mol_type = other RNA
gacacgcagagggacccaga

SEQ ID NO: 9481 - RNA, 20 nt, synthetic construct
  source 1..20: mol_type = other RNA
gacaagcagagacacgcaga

SEQ ID NO: 9482 - RNA, 20 nt, synthetic construct
  source 1..20: mol_type = other RNA
ggacaagcagagacacgcag

SEQ ID NO: 9483 - RNA, 20 nt, synthetic construct
  source 1..20: mol_type = other RNA
gtcactgacacacacaggct

SEQ ID NO: 9484 - RNA, 20 nt, synthetic construct
  source 1..20: mol_type = other RNA
tagacgtcactgacacacac

SEQ ID NO: 9485 - RNA, 20 nt, synthetic construct
  source 1..20: mol_type = other RNA
tgtgtgtgtgtccttgtccg

SEQ ID NO: 9486 - RNA, 20 nt, synthetic construct
  source 1..20: mol_type = other RNA
tccgaggagccgagagagtg

SEQ ID NO: 9487 - RNA, 20 nt, synthetic construct
  source 1..20: mol_type = other RNA
ccgaggagccgagagagtga

SEQ ID NO: 9488 - RNA, 20 nt, synthetic construct
  source 1..20: mol_type = other RNA
cgaggagccgagagagtgag

SEQ ID NO: 9489 - RNA, 20 nt, synthetic construct
  source 1..20: mol_type = other RNA
gaggagccgagagagtgagg

SEQ ID NO: 9490 - RNA, 20 nt, synthetic construct
  source 1..20: mol_type = other RNA
ccctcactctctcggctcct

SEQ ID NO: 9491 - RNA, 20 nt, synthetic construct
  source 1..20: mol_type = other RNA
gagagagtgagggggaatga

SEQ ID NO: 9492 - RNA, 20 nt, synthetic construct
  source 1..20: mol_type = other RNA
agagagtgagggggaatgaa

SEQ ID NO: 9493 - RNA, 20 nt, synthetic construct
  source 1..20: mol_type = other RNA
ttcattccccctcactctct

SEQ ID NO: 9494 - RNA, 20 nt, synthetic construct
  source 1..20: mol_type = other RNA
tgagggggaatgaagggcca

SEQ ID NO: 9495 - RNA, 20 nt, synthetic construct
  source 1..20: mol_type = other RNA
gggggaatgaagggccaagg

SEQ ID NO: 9496 - RNA, 20 nt, synthetic construct
  source 1..20: mol_type = other RNA
aatgaagggccaaggaggcc

SEQ ID NO: 9497 - RNA, 20 nt, synthetic construct
  source 1..20: mol_type = other RNA
aagggccaaggaggcctggc

SEQ ID NO: 9498 - RNA, 20 nt, synthetic construct
  source 1..20: mol_type = other RNA
agggccaaggaggcctggct

SEQ ID NO: 9499 - RNA, 20 nt, synthetic construct
  source 1..20: mol_type = other RNA
gggccaaggaggcctggctg

SEQ ID NO: 9500 - RNA, 20 nt, synthetic construct
  source 1..20: mol_type = other RNA
caaggaggcctggctggggc

SEQ ID NO: 9501 - RNA, 20 nt, synthetic construct
  source 1..20: mol_type = other RNA
aaggaggcctggctggggct

SEQ ID NO: 9502 - RNA, 20 nt, synthetic construct
  source 1..20: mol_type = other RNA
cagccccagccaggcctcct

SEQ ID NO: 9503 - RNA, 20 nt, synthetic construct
  source 1..20: mol_type = other RNA
aggcctggctggggctgggc

SEQ ID NO: 9504 - RNA, 20 nt, synthetic construct
  source 1..20: mol_type = other RNA
ggcctggctggggctgggct

SEQ ID NO: 9505 - RNA, 20 nt, synthetic construct
  source 1..20: mol_type = other RNA
gcctggctggggctgggctg

SEQ ID NO: 9506 - RNA, 20 nt, synthetic construct
  source 1..20: mol_type = other RNA
cctggctggggctgggctgg

SEQ ID NO: 9507 - RNA, 20 nt, synthetic construct
  source 1..20: mol_type = other RNA
ggctggggctgggctggggg

SEQ ID NO: 9508 - RNA, 20 nt, synthetic construct
  source 1..20: mol_type = other RNA
cccccagcccagccccagcc

SEQ ID NO: 9509 - RNA, 20 nt, synthetic construct
  source 1..20: mol_type = other RNA
tggggctgggctgggggtgg

SEQ ID NO: 9510 - RNA, 20 nt, synthetic construct
  source 1..20: mol_type = other RNA
ggctgggctgggggtggagg

SEQ ID NO: 9511 - RNA, 20 nt, synthetic construct
  source 1..20: mol_type = other RNA
gctgggctgggggtggaggc

SEQ ID NO: 9512 - RNA, 20 nt, synthetic construct
  source 1..20: mol_type = other RNA
ctgggctgggggtggaggcg

SEQ ID NO: 9513 - RNA, 20 nt, synthetic construct
  source 1..20: mol_type = other RNA
ctgggggtggaggcggggag

SEQ ID NO: 9514 - RNA, 20 nt, synthetic construct
  source 1..20: mol_type = other RNA
tgggggtggaggcggggaga

SEQ ID NO: 9515 - RNA, 20 nt, synthetic construct
  source 1..20: mol_type = other RNA
gggggtggaggcggggagag

SEQ ID NO: 9516 - RNA, 20 nt, synthetic construct
  source 1..20: mol_type = other RNA
aggcggggagaggggcgtca

SEQ ID NO: 9517 - RNA, 20 nt, synthetic construct
  source 1..20: mol_type = other RNA
gcgtcacggcctgagctgag

SEQ ID NO: 9518 - RNA, 20 nt, synthetic construct
  source 1..20: mol_type = other RNA
cgtcacggcctgagctgaga

SEQ ID NO: 9519 - RNA, 20 nt, synthetic construct
  source 1..20: mol_type = other RNA
gtcacggcctgagctgagag

SEQ ID NO: 9520 - RNA, 20 nt, synthetic construct
  source 1..20: mol_type = other RNA
ggcctgagctgagaggggag

SEQ ID NO: 9521 - RNA, 20 nt, synthetic construct
  source 1..20: mol_type = other RNA
ctccactcccctctcagctc

SEQ ID NO: 9522 - RNA, 20 nt, synthetic construct
  source 1..20: mol_type = other RNA
ctgagaggggagtggagttc

SEQ ID NO: 9523 - RNA, 20 nt, synthetic construct
  source 1..20: mol_type = other RNA
agaggggagtggagttctgg

SEQ ID NO: 9524 - RNA, 20 nt, synthetic construct
  source 1..20: mol_type = other RNA
ttaccagacacagagcccag

SEQ ID NO: 9525 - RNA, 20 nt, synthetic construct
  source 1..20: mol_type = other RNA
taccagacacagagcccaga

SEQ ID NO: 9526 - RNA, 20 nt, synthetic construct
  source 1..20: mol_type = other RNA
gtccctctgggctctgtgtc

SEQ ID NO: 9527 - RNA, 20 nt, synthetic construct
  source 1..20: mol_type = other RNA
gagggacagcgcccagagcc

SEQ ID NO: 9528 - RNA, 20 nt, synthetic construct
  source 1..20: mol_type = other RNA
gctctgggcgctgtccctct

SEQ ID NO: 9529 - RNA, 20 nt, synthetic construct
  source 1..20: mol_type = other RNA
ggctctgggcgctgtccctc

SEQ ID NO: 9530 - RNA, 20 nt, synthetic construct
  source 1..20: mol_type = other RNA
agagcccggatagagagaca

SEQ ID NO: 9531 - RNA, 20 nt, synthetic construct
  source 1..20: mol_type = other RNA
tgtctctctatccgggctct

SEQ ID NO: 9532 - RNA, 20 nt, synthetic construct
  source 1..20: mol_type = other RNA
gtgtctctctatccgggctc

SEQ ID NO: 9533 - RNA, 20 nt, synthetic construct
  source 1..20: mol_type = other RNA
gaggccgtgtctctctatcc

SEQ ID NO: 9534 - RNA, 20 nt, synthetic construct
  source 1..20: mol_type = other RNA
tgaggccgtgtctctctatc

SEQ ID NO: 9535 - RNA, 20 nt, synthetic construct
  source 1..20: mol_type = other RNA
agacacggcctcactggctc

SEQ ID NO: 9536 - RNA, 20 nt, synthetic construct
  source 1..20: mol_type = other RNA
cggcctcactggctcaggac

SEQ ID NO: 9537 - RNA, 20 nt, synthetic construct
  source 1..20: mol_type = other RNA
ggcctcactggctcaggaca

SEQ ID NO: 9538 - RNA, 20 nt, synthetic construct
  source 1..20: mol_type = other RNA
gcctcactggctcaggacag

SEQ ID NO: 9539 - RNA, 20 nt, synthetic construct
  source 1..20: mol_type = other RNA
cctcactggctcaggacagg

SEQ ID NO: 9540 - RNA, 20 nt, synthetic construct
  source 1..20: mol_type = other RNA
ccccctgtcctgagccagtg

SEQ ID NO: 9541 - RNA, 20 nt, synthetic construct
  source 1..20: mol_type = other RNA
ggacagggggcacagccacc

SEQ ID NO: 9542 - RNA, 20 nt, synthetic construct
  source 1..20: mol_type = other RNA
gacagggggcacagccacca

SEQ ID NO: 9543 - RNA, 20 nt, synthetic construct
  source 1..20: mol_type = other RNA
gagggggaaggggaccctgg

SEQ ID NO: 9544 - RNA, 20 nt, synthetic construct
  source 1..20: mol_type = other RNA
gaggagggggaaggggaccc

SEQ ID NO: 9545 - RNA, 20 nt, synthetic construct
  source 1..20: mol_type = other RNA
gggagctgaggagggggaag

SEQ ID NO: 9546 - RNA, 20 nt, synthetic construct
  source 1..20: mol_type = other RNA
agggagctgaggagggggaa

SEQ ID NO: 9547 - RNA, 20 nt, synthetic construct
  source 1..20: mol_type = other RNA
gagggagctgaggaggggga

SEQ ID NO: 9548 - RNA, 20 nt, synthetic construct
  source 1..20: mol_type = other RNA
cagggagggagctgaggagg

SEQ ID NO: 9549 - RNA, 20 nt, synthetic construct
  source 1..20: mol_type = other RNA
ccagggagggagctgaggag

SEQ ID NO: 9550 - RNA, 20 nt, synthetic construct
  source 1..20: mol_type = other RNA
gccagggagggagctgagga

SEQ ID NO: 9551 - RNA, 20 nt, synthetic construct
  source 1..20: mol_type = other RNA
ggccagggagggagctgagg

SEQ ID NO: 9552 - RNA, 20 nt, synthetic construct
  source 1..20: mol_type = other RNA
aggggccagggagggagctg

SEQ ID NO: 9553 - RNA, 20 nt, synthetic construct
  source 1..20: mol_type = other RNA
tttcttaaaggggccaggga

SEQ ID NO: 9554 - RNA, 20 nt, synthetic construct
  source 1..20: mol_type = other RNA
ctttcttaaaggggccaggg

SEQ ID NO: 9555 - RNA, 20 nt, synthetic construct
  source 1..20: mol_type = other RNA
gctctttcttaaaggggcca

SEQ ID NO: 9556 - RNA, 20 nt, synthetic construct
  source 1..20: mol_type = other RNA
agctctttcttaaaggggcc

SEQ ID NO: 9557 - RNA, 20 nt, synthetic construct
  source 1..20: mol_type = other RNA
ggatcagctctttcttaaag

SEQ ID NO: 9558 - RNA, 20 nt, synthetic construct
  source 1..20: mol_type = other RNA
aggatcagctctttcttaaa

SEQ ID NO: 9559 - RNA, 20 nt, synthetic construct
  source 1..20: mol_type = other RNA
gaggatcagctctttcttaa

SEQ ID NO: 9560 - RNA, 20 nt, synthetic construct
  source 1..20: mol_type = other RNA
gggttaactcaagagaggag

SEQ ID NO: 9561 - RNA, 20 nt, synthetic construct
  source 1..20: mol_type = other RNA
atcaggggttaactcaagag

SEQ ID NO: 9562 - RNA, 20 nt, synthetic construct
  source 1..20: mol_type = other RNA
gagttaacccctgattgtcc

SEQ ID NO: 9563 - RNA, 20 nt, synthetic construct
  source 1..20: mol_type = other RNA
ttaacccctgattgtccagg

SEQ ID NO: 9564 - RNA, 20 nt, synthetic construct
  source 1..20: mol_type = other RNA
ctgattgtccaggtggcccc

SEQ ID NO: 9565 - RNA, 20 nt, synthetic construct
  source 1..20: mol_type = other RNA
tgattgtccaggtggcccct

SEQ ID NO: 9566 - RNA, 20 nt, synthetic construct
  source 1..20: mol_type = other RNA
ggggccacctggacaatcag

SEQ ID NO: 9567 - RNA, 20 nt, synthetic construct
  source 1..20: mol_type = other RNA
aggggccacctggacaatca

SEQ ID NO: 9568 - RNA, 20 nt, synthetic construct
  source 1..20: mol_type = other RNA
caggggccacctggacaatc

SEQ ID NO: 9569 - RNA, 20 nt, synthetic construct
  source 1..20: mol_type = other RNA
tccaggtggcccctgggctc

SEQ ID NO: 9570 - RNA, 20 nt, synthetic construct
  source 1..20: mol_type = other RNA
tggcccctgggctctggccc

SEQ ID NO: 9571 - RNA, 20 nt, synthetic construct
  source 1..20: mol_type = other RNA
cccctgggctctggccctgg

SEQ ID NO: 9572 - RNA, 20 nt, synthetic construct
  source 1..20: mol_type = other RNA
ccctgggctctggccctggt

SEQ ID NO: 9573 - RNA, 20 nt, synthetic construct
  source 1..20: mol_type = other RNA
tgggctctggccctggtggg

SEQ ID NO: 9574 - RNA, 20 nt, synthetic construct
  source 1..20: mol_type = other RNA
ccaccagggccagagcccag

SEQ ID NO: 9575 - RNA, 20 nt, synthetic construct
  source 1..20: mol_type = other RNA
cccaccagggccagagccca

SEQ ID NO: 9576 - RNA, 20 nt, synthetic construct
  source 1..20: mol_type = other RNA
gctctggccctggtgggcgg

SEQ ID NO: 9577 - RNA, 20 nt, synthetic construct
  source 1..20: mol_type = other RNA
gccctggtgggcggaggcaa

SEQ ID NO: 9578 - RNA, 20 nt, synthetic construct
  source 1..20: mol_type = other RNA
ccctggtgggcggaggcaaa

SEQ ID NO: 9579 - RNA, 20 nt, synthetic construct
  source 1..20: mol_type = other RNA
cctggtgggcggaggcaaag

SEQ ID NO: 9580 - RNA, 20 nt, synthetic construct
  source 1..20: mol_type = other RNA
ctggtgggcggaggcaaagg

SEQ ID NO: 9581 - RNA, 20 nt, synthetic construct
  source 1..20: mol_type = other RNA
ccctttgcctccgcccacca

SEQ ID NO: 9582 - RNA, 20 nt, synthetic construct
  source 1..20: mol_type = other RNA
cccctttgcctccgcccacc

SEQ ID NO: 9583 - RNA, 20 nt, synthetic construct
  source 1..20: mol_type = other RNA
gcggaggcaaagggggagcc

SEQ ID NO: 9584 - RNA, 20 nt, synthetic construct
  source 1..20: mol_type = other RNA
cggaggcaaagggggagcca

SEQ ID NO: 9585 - RNA, 20 nt, synthetic construct
  source 1..20: mol_type = other RNA
ggaggcaaagggggagccag

SEQ ID NO: 9586 - RNA, 20 nt, synthetic construct
  source 1..20: mol_type = other RNA
ggcaaagggggagccagggg

SEQ ID NO: 9587 - RNA, 20 nt, synthetic construct
  source 1..20: mol_type = other RNA
ggggagccaggggcggagaa

SEQ ID NO: 9588 - RNA, 20 nt, synthetic construct
  source 1..20: mol_type = other RNA
gggagccaggggcggagaaa

SEQ ID NO: 9589 - RNA, 20 nt, synthetic construct
  source 1..20: mol_type = other RNA
ggcaaccctttctccgcccc

SEQ ID NO: 9590 - RNA, 20 nt, synthetic construct
  source 1..20: mol_type = other RNA
gagaaagggttgcccaagtc

SEQ ID NO: 9591 - RNA, 20 nt, synthetic construct
  source 1..20: mol_type = other RNA
agaaagggttgcccaagtct

SEQ ID NO: 9592 - RNA, 20 nt, synthetic construct
  source 1..20: mol_type = other RNA
gttgcccaagtctgggagtg

SEQ ID NO: 9593 - RNA, 20 nt, synthetic construct
  source 1..20: mol_type = other RNA
ttgcccaagtctgggagtga

SEQ ID NO: 9594 - RNA, 20 nt, synthetic construct
  source 1..20: mol_type = other RNA
ccaagtctgggagtgaggga

SEQ ID NO: 9595 - RNA, 20 nt, synthetic construct
  source 1..20: mol_type = other RNA
agtctgggagtgagggaagg

SEQ ID NO: 9596 - RNA, 20 nt, synthetic construct
  source 1..20: mol_type = other RNA
cttccctcactcccagactt

SEQ ID NO: 9597 - RNA, 20 nt, synthetic construct
  source 1..20: mol_type = other RNA
ccttccctcactcccagact

SEQ ID NO: 9598 - RNA, 20 nt, synthetic construct
  source 1..20: mol_type = other RNA
tgggagtgagggaaggaggc

SEQ ID NO: 9599 - RNA, 20 nt, synthetic construct
  source 1..20: mol_type = other RNA
gggagtgagggaaggaggca

SEQ ID NO: 9600 - RNA, 20 nt, synthetic construct
  source 1..20: mol_type = other RNA
ggagtgagggaaggaggcag

SEQ ID NO: 9601 - RNA, 20 nt, synthetic construct
  source 1..20: mol_type = other RNA
aggaggcaggggtgctgaga

SEQ ID NO: 9602 - RNA, 20 nt, synthetic construct
  source 1..20: mol_type = other RNA
aggcaggggtgctgagaagg

SEQ ID NO: 9603 - RNA, 20 nt, synthetic construct
  source 1..20: mol_type = other RNA
ggtgctgagaaggcggctgc

SEQ ID NO: 9604 - RNA, 20 nt, synthetic construct
  source 1..20: mol_type = other RNA
gtgctgagaaggcggctgct

SEQ ID NO: 9605 - RNA, 20 nt, synthetic construct
  source 1..20: mol_type = other RNA
aggcggctgctgggcagagc

SEQ ID NO: 9606 - RNA, 20 nt, synthetic construct
  source 1..20: mol_type = other RNA
cggctgctgggcagagccgg

SEQ ID NO: 9607 - RNA, 20 nt, synthetic construct
  source 1..20: mol_type = other RNA
gctgggcagagccggtggca

SEQ ID NO: 9608 - RNA, 20 nt, synthetic construct
  source 1..20: mol_type = other RNA
ctgggcagagccggtggcaa

SEQ ID NO: 9609 - RNA, 20 nt, synthetic construct
  source 1..20: mol_type = other RNA
gcaggggaggcccttgccac

SEQ ID NO: 9610 - RNA, 20 nt, synthetic construct
  source 1..20: mol_type = other RNA
gcctcccctgccgctgtgcc

SEQ ID NO: 9611 - RNA, 20 nt, synthetic construct
  source 1..20: mol_type = other RNA
cccctgccgctgtgccaggc

SEQ ID NO: 9612 - RNA, 20 nt, synthetic construct
  source 1..20: mol_type = other RNA
gcctggcacagcggcagggg

SEQ ID NO: 9613 - RNA, 20 nt, synthetic construct
  source 1..20: mol_type = other RNA
cctgcctggcacagcggcag

SEQ ID NO: 9614 - RNA, 20 nt, synthetic construct
  source 1..20: mol_type = other RNA
gcctgcctggcacagcggca

SEQ ID NO: 9615 - RNA, 20 nt, synthetic construct
  source 1..20: mol_type = other RNA
tgcctgcctggcacagcggc

SEQ ID NO: 9616 - RNA, 20 nt, synthetic construct
  source 1..20: mol_type = other RNA
gcactgcctgcctggcacag

SEQ ID NO: 9617 - RNA, 20 nt, synthetic construct
  source 1..20: mol_type = other RNA
caggcaggcagtgccaaatc

SEQ ID NO: 9618 - RNA, 20 nt, synthetic construct
  source 1..20: mol_type = other RNA
aggcaggcagtgccaaatcc

SEQ ID NO: 9619 - RNA, 20 nt, synthetic construct
  source 1..20: mol_type = other RNA
ggcaggcagtgccaaatccg

SEQ ID NO: 9620 - RNA, 20 nt, synthetic construct
  source 1..20: mol_type = other RNA
cggatttggcactgcctgcc

SEQ ID NO: 9621 - RNA, 20 nt, synthetic construct
  source 1..20: mol_type = other RNA
agtgccaaatccggggagcc

SEQ ID NO: 9622 - RNA, 20 nt, synthetic construct
  source 1..20: mol_type = other RNA
aaatccggggagcctggagc

SEQ ID NO: 9623 - RNA, 20 nt, synthetic construct
  source 1..20: mol_type = other RNA
aatccggggagcctggagct

SEQ ID NO: 9624 - RNA, 20 nt, synthetic construct
  source 1..20: mol_type = other RNA
atccggggagcctggagctg

SEQ ID NO: 9625 - RNA, 20 nt, synthetic construct
  source 1..20: mol_type = other RNA
agctccaggctccccggatt

SEQ ID NO: 9626 - RNA, 20 nt, synthetic construct
  source 1..20: mol_type = other RNA
ccggggagcctggagctggg

SEQ ID NO: 9627 - RNA, 20 nt, synthetic construct
  source 1..20: mol_type = other RNA
gggagcctggagctgggggg

SEQ ID NO: 9628 - RNA, 20 nt, synthetic construct
  source 1..20: mol_type = other RNA
ggagcctggagctgggggga

SEQ ID NO: 9629 - RNA, 20 nt, synthetic construct
  source 1..20: mol_type = other RNA
ccccccagctccaggctccc

SEQ ID NO: 9630 - RNA, 20 nt, synthetic construct
  source 1..20: mol_type = other RNA
cctggagctggggggagggc

SEQ ID NO: 9631 - RNA, 20 nt, synthetic construct
  source 1..20: mol_type = other RNA
ctggagctggggggagggcc

SEQ ID NO: 9632 - RNA, 20 nt, synthetic construct
  source 1..20: mol_type = other RNA
tggagctggggggagggccg

SEQ ID NO: 9633 - RNA, 20 nt, synthetic construct
  source 1..20: mol_type = other RNA
ccggccctccccccagctcc

SEQ ID NO: 9634 - RNA, 20 nt, synthetic construct
  source 1..20: mol_type = other RNA
ggggagggccggggacagcc

SEQ ID NO: 9635 - RNA, 20 nt, synthetic construct
  source 1..20: mol_type = other RNA
gggcagggccgggctgtccc

SEQ ID NO: 9636 - RNA, 20 nt, synthetic construct
  source 1..20: mol_type = other RNA
ggccctgccccctcccccgc

SEQ ID NO: 9637 - RNA, 20 nt, synthetic construct
  source 1..20: mol_type = other RNA
gccctgccccctcccccgct

SEQ ID NO: 9638 - RNA, 20 nt, synthetic construct
  source 1..20: mol_type = other RNA
gcgggggagggggcagggcc

SEQ ID NO: 9639 - RNA, 20 nt, synthetic construct
  source 1..20: mol_type = other RNA
agcgggggagggggcagggc

SEQ ID NO: 9640 - RNA, 20 nt, synthetic construct
  source 1..20: mol_type = other RNA
tcccagcgggggagggggca

SEQ ID NO: 9641 - RNA, 20 nt, synthetic construct
  source 1..20: mol_type = other RNA
ctcccagcgggggagggggc

SEQ ID NO: 9642 - RNA, 20 nt, synthetic construct
  source 1..20: mol_type = other RNA
tgggctcccagcgggggagg

SEQ ID NO: 9643 - RNA, 20 nt, synthetic construct
  source 1..20: mol_type = other RNA
ttgggctcccagcgggggag

SEQ ID NO: 9644 - RNA, 20 nt, synthetic construct
  source 1..20: mol_type = other RNA
gttgggctcccagcggggga

SEQ ID NO: 9645 - RNA, 20 nt, synthetic construct
  source 1..20: mol_type = other RNA
tgttgggctcccagcggggg

SEQ ID NO: 9646 - RNA, 20 nt, synthetic construct
  source 1..20: mol_type = other RNA
agttgttgggctcccagcgg

SEQ ID NO: 9647 - RNA, 20 nt, synthetic construct
  source 1..20: mol_type = other RNA
aagttgttgggctcccagcg

SEQ ID NO: 9648 - RNA, 20 nt, synthetic construct
  source 1..20: mol_type = other RNA
gaagttgttgggctcccagc

SEQ ID NO: 9649 - RNA, 20 nt, synthetic construct
  source 1..20: mol_type = other RNA
agaagttgttgggctcccag

SEQ ID NO: 9650 - RNA, 20 nt, synthetic construct
  source 1..20: mol_type = other RNA
aacaacttctgaggaaagtt

SEQ ID NO: 9651 - RNA, 20 nt, synthetic construct
  source 1..20: mol_type = other RNA
aactttcctcagaagttgtt

SEQ ID NO: 9652 - RNA, 20 nt, synthetic construct
  source 1..20: mol_type = other RNA
aaactttcctcagaagttgt

SEQ ID NO: 9653 - RNA, 20 nt, synthetic construct
  source 1..20: mol_type = other RNA
tgaggaaagtttggcaccca

SEQ ID NO: 9654 - RNA, 20 nt, synthetic construct
  source 1..20: mol_type = other RNA
aaagtttggcacccatggcg

SEQ ID NO: 9655 - RNA, 20 nt, synthetic construct
  source 1..20: mol_type = other RNA
gtttggcacccatggcgtgg

SEQ ID NO: 9656 - RNA, 20 nt, synthetic construct
  source 1..20: mol_type = other RNA
ccatggcgtggcggtgcccc

SEQ ID NO: 9657 - RNA, 20 nt, synthetic construct
  source 1..20: mol_type = other RNA
ctggggcaccgccacgccat

SEQ ID NO: 9658 - RNA, 20 nt, synthetic construct
  source 1..20: mol_type = other RNA
cctggggcaccgccacgcca

SEQ ID NO: 9659 - RNA, 20 nt, synthetic construct
  source 1..20: mol_type = other RNA
ggcggtgccccaggatgggc

SEQ ID NO: 9660 - RNA, 20 nt, synthetic construct
  source 1..20: mol_type = other RNA
gcggtgccccaggatgggca

SEQ ID NO: 9661 - RNA, 20 nt, synthetic construct
  source 1..20: mol_type = other RNA
caggatgggcagggtcccgc

SEQ ID NO: 9662 - RNA, 20 nt, synthetic construct
  source 1..20: mol_type = other RNA
gcgggaccctgcccatcctg

SEQ ID NO: 9663 - RNA, 20 nt, synthetic construct
  source 1..20: mol_type = other RNA
agcgggaccctgcccatcct

SEQ ID NO: 9664 - RNA, 20 nt, synthetic construct
  source 1..20: mol_type = other RNA
cagcgggaccctgcccatcc

SEQ ID NO: 9665 - RNA, 20 nt, synthetic construct
  source 1..20: mol_type = other RNA
tgggcagggtcccgctggcc

SEQ ID NO: 9666 - RNA, 20 nt, synthetic construct
  source 1..20: mol_type = other RNA
ggtcccgctggcctggtgct

SEQ ID NO: 9667 - RNA, 20 nt, synthetic construct
  source 1..20: mol_type = other RNA
gcgccaagcaccaggccagc

SEQ ID NO: 9668 - RNA, 20 nt, synthetic construct
  source 1..20: mol_type = other RNA
agcgccaagcaccaggccag

SEQ ID NO: 9669 - RNA, 20 nt, synthetic construct
  source 1..20: mol_type = other RNA
gcctggtgcttggcgctgtg

SEQ ID NO: 9670 - RNA, 20 nt, synthetic construct
  source 1..20: mol_type = other RNA
ggtgcttggcgctgtgcggc

SEQ ID NO: 9671 - RNA, 20 nt, synthetic construct
  source 1..20: mol_type = other RNA
gtgcttggcgctgtgcggct

SEQ ID NO: 9672 - RNA, 20 nt, synthetic construct
  source 1..20: mol_type = other RNA
gccgcacagcgccaagcacc

SEQ ID NO: 9673 - RNA, 20 nt, synthetic construct
  source 1..20: mol_type = other RNA
gctgtgcggctgggcgtgca

SEQ ID NO: 9674 - RNA, 20 nt, synthetic construct
  source 1..20: mol_type = other RNA
gctgggcgtgcatggccccc

SEQ ID NO: 9675 - RNA, 20 nt, synthetic construct
  source 1..20: mol_type = other RNA
ctgggcgtgcatggccccca

SEQ ID NO: 9676 - RNA, 20 nt, synthetic construct
  source 1..20: mol_type = other RNA
tgggcgtgcatggcccccag

SEQ ID NO: 9677 - RNA, 20 nt, synthetic construct
  source 1..20: mol_type = other RNA
tggcccccaggggtgagtga

SEQ ID NO: 9678 - RNA, 20 nt, synthetic construct
  source 1..20: mol_type = other RNA
ggcccccaggggtgagtgat

SEQ ID NO: 9679 - RNA, 20 nt, synthetic construct
  source 1..20: mol_type = other RNA
gcccccaggggtgagtgatg

SEQ ID NO: 9680 - RNA, 20 nt, synthetic construct
  source 1..20: mol_type = other RNA
cccccaggggtgagtgatgg

SEQ ID NO: 9681 - RNA, 20 nt, synthetic construct
  source 1..20: mol_type = other RNA
cccccatcactcacccctgg

SEQ ID NO: 9682 - RNA, 20 nt, synthetic construct
  source 1..20: mol_type = other RNA
gcccccatcactcacccctg

SEQ ID NO: 9683 - RNA, 20 nt, synthetic construct
  source 1..20: mol_type = other RNA
agcccccatcactcacccct

SEQ ID NO: 9684 - RNA, 20 nt, synthetic construct
  source 1..20: mol_type = other RNA
gagcccccatcactcacccc

SEQ ID NO: 9685 - RNA, 20 nt, synthetic construct
  source 1..20: mol_type = other RNA
gtgagtgatgggggctcctt

SEQ ID NO: 9686 - RNA, 20 nt, synthetic construct
  source 1..20: mol_type = other RNA
tgagtgatgggggctccttg

SEQ ID NO: 9687 - RNA, 20 nt, synthetic construct
  source 1..20: mol_type = other RNA
tgatgggggctccttggggc

SEQ ID NO: 9688 - RNA, 20 nt, synthetic construct
  source 1..20: mol_type = other RNA
gatgggggctccttggggca

SEQ ID NO: 9689 - RNA, 20 nt, synthetic construct
  source 1..20: mol_type = other RNA
ccttggggcagggatcccct

SEQ ID NO: 9690 - RNA, 20 nt, synthetic construct
  source 1..20: mol_type = other RNA
tggggcagggatcccctcgg

SEQ ID NO: 9691 - RNA, 20 nt, synthetic construct
  source 1..20: mol_type = other RNA
ggggcagggatcccctcgga

SEQ ID NO: 9692 - RNA, 20 nt, synthetic construct
  source 1..20: mol_type = other RNA
gggcagggatcccctcggag

SEQ ID NO: 9693 - RNA, 20 nt, synthetic construct
  source 1..20: mol_type = other RNA
agggatcccctcggaggggc

SEQ ID NO: 9694 - RNA, 20 nt, synthetic construct
  source 1..20: mol_type = other RNA
gggatcccctcggaggggct

SEQ ID NO: 9695 - RNA, 20 nt, synthetic construct
  source 1..20: mol_type = other RNA
ggatcccctcggaggggctg

SEQ ID NO: 9696 - RNA, 20 nt, synthetic construct
  source 1..20: mol_type = other RNA
cccctcggaggggctggggc

SEQ ID NO: 9697 - RNA, 20 nt, synthetic construct
  source 1..20: mol_type = other RNA
ccctcggaggggctggggca

SEQ ID NO: 9698 - RNA, 20 nt, synthetic construct
  source 1..20: mol_type = other RNA
cctcggaggggctggggcag

SEQ ID NO: 9699 - RNA, 20 nt, synthetic construct
  source 1..20: mol_type = other RNA
cctgccccagcccctccgag

SEQ ID NO: 9700 - RNA, 20 nt, synthetic construct
  source 1..20: mol_type = other RNA
ccctgccccagcccctccga

SEQ ID NO: 9701 - RNA, 20 nt, synthetic construct
  source 1..20: mol_type = other RNA
cccctgccccagcccctccg

SEQ ID NO: 9702 - RNA, 20 nt, synthetic construct
  source 1..20: mol_type = other RNA
ggggctggggcaggggtagg

SEQ ID NO: 9703 - RNA, 20 nt, synthetic construct
  source 1..20: mol_type = other RNA
gctggggcaggggtaggagg

SEQ ID NO: 9704 - RNA, 20 nt, synthetic construct
  source 1..20: mol_type = other RNA
ctggggcaggggtaggaggt

SEQ ID NO: 9705 - RNA, 20 nt, synthetic construct
  source 1..20: mol_type = other RNA
tggggcaggggtaggaggtg

SEQ ID NO: 9706 - RNA, 20 nt, synthetic construct
  source 1..20: mol_type = other RNA
ggggcaggggtaggaggtgg

SEQ ID NO: 9707 - RNA, 20 nt, synthetic construct
  source 1..20: mol_type = other RNA
gggtaggaggtgggggatga

SEQ ID NO: 9708 - RNA, 20 nt, synthetic construct
  source 1..20: mol_type = other RNA
aggaggtgggggatgatggc

SEQ ID NO: 9709 - RNA, 20 nt, synthetic construct
  source 1..20: mol_type = other RNA
gtgggggatgatggcaggtg

SEQ ID NO: 9710 - RNA, 20 nt, synthetic construct
  source 1..20: mol_type = other RNA
tgggggatgatggcaggtgt

SEQ ID NO: 9711 - RNA, 20 nt, synthetic construct
  source 1..20: mol_type = other RNA
gggggatgatggcaggtgtg

SEQ ID NO: 9712 - RNA, 20 nt, synthetic construct
  source 1..20: mol_type = other RNA
ggggatgatggcaggtgtgg

SEQ ID NO: 9713 - RNA, 20 nt, synthetic construct
  source 1..20: mol_type = other RNA
gggatgatggcaggtgtggg

SEQ ID NO: 9714 - RNA, 20 nt, synthetic construct
  source 1..20: mol_type = other RNA
gatggcaggtgtggggggcc

SEQ ID NO: 9715 - RNA, 20 nt, synthetic construct
  source 1..20: mol_type = other RNA
atggcaggtgtggggggcct

SEQ ID NO: 9716 - RNA, 20 nt, synthetic construct
  source 1..20: mol_type = other RNA
caggtgtggggggcctgggc

SEQ ID NO: 9717 - RNA, 20 nt, synthetic construct
  source 1..20: mol_type = other RNA
tggggggcctgggctggctt

SEQ ID NO: 9718 - RNA, 20 nt, synthetic construct
  source 1..20: mol_type = other RNA
ggggggcctgggctggctta

SEQ ID NO: 9719 - RNA, 20 nt, synthetic construct
  source 1..20: mol_type = other RNA
gctggcttagggagtttcct

SEQ ID NO: 9720 - RNA, 20 nt, synthetic construct
  source 1..20: mol_type = other RNA
ctggcttagggagtttcctt

SEQ ID NO: 9721 - RNA, 20 nt, synthetic construct
  source 1..20: mol_type = other RNA
atgtcggcctaagggcctgg

SEQ ID NO: 9722 - RNA, 20 nt, synthetic construct
  source 1..20: mol_type = other RNA
tgtcggcctaagggcctggc

SEQ ID NO: 9723 - RNA, 20 nt, synthetic construct
  source 1..20: mol_type = other RNA
gtcggcctaagggcctggcg

SEQ ID NO: 9724 - RNA, 20 nt, synthetic construct
  source 1..20: mol_type = other RNA
ctaagggcctggcggggtcc

SEQ ID NO: 9725 - RNA, 20 nt, synthetic construct
  source 1..20: mol_type = other RNA
caggaccccgccaggccctt

SEQ ID NO: 9726 - RNA, 20 nt, synthetic construct
  source 1..20: mol_type = other RNA
cctggcggggtcctggccgc

SEQ ID NO: 9727 - RNA, 20 nt, synthetic construct
  source 1..20: mol_type = other RNA
ggcggggtcctggccgccgg

SEQ ID NO: 9728 - RNA, 20 nt, synthetic construct
  source 1..20: mol_type = other RNA
gcggggtcctggccgccggt

SEQ ID NO: 9729 - RNA, 20 nt, synthetic construct
  source 1..20: mol_type = other RNA
ccggcggccaggaccccgcc

SEQ ID NO: 9730 - RNA, 20 nt, synthetic construct
  source 1..20: mol_type = other RNA
ggtcctggccgccggtgggc

SEQ ID NO: 9731 - RNA, 20 nt, synthetic construct
  source 1..20: mol_type = other RNA
tggccgccggtgggcaggca

SEQ ID NO: 9732 - RNA, 20 nt, synthetic construct
  source 1..20: mol_type = other RNA
ttgcctgcccaccggcggcc

SEQ ID NO: 9733 - RNA, 20 nt, synthetic construct
  source 1..20: mol_type = other RNA
gccggtgggcaggcaaggac

SEQ ID NO: 9734 - RNA, 20 nt, synthetic construct
  source 1..20: mol_type = other RNA
ccggtgggcaggcaaggaca

SEQ ID NO: 9735 - RNA, 20 nt, synthetic construct
  source 1..20: mol_type = other RNA
tgtccttgcctgcccaccgg

SEQ ID NO: 9736 - RNA, 20 nt, synthetic construct
  source 1..20: mol_type = other RNA
gtgggcaggcaaggacaggg

SEQ ID NO: 9737 - RNA, 20 nt, synthetic construct
  source 1..20: mol_type = other RNA
ccctgtccttgcctgcccac

SEQ ID NO: 9738 - RNA, 20 nt, synthetic construct
  source 1..20: mol_type = other RNA
gcaaggacagggtggaactg

SEQ ID NO: 9739 - RNA, 20 nt, synthetic construct
  source 1..20: mol_type = other RNA
caaggacagggtggaactga

SEQ ID NO: 9740 - RNA, 20 nt, synthetic construct
  source 1..20: mol_type = other RNA
gacagggtggaactgagggc

SEQ ID NO: 9741 - RNA, 20 nt, synthetic construct
  source 1..20: mol_type = other RNA
gggtggaactgagggccgga

SEQ ID NO: 9742 - RNA, 20 nt, synthetic construct
  source 1..20: mol_type = other RNA
aactgagggccggaaggagc

SEQ ID NO: 9743 - RNA, 20 nt, synthetic construct
  source 1..20: mol_type = other RNA
actgagggccggaaggagct

SEQ ID NO: 9744 - RNA, 20 nt, synthetic construct
  source 1..20: mol_type = other RNA
ctgagggccggaaggagctg

SEQ ID NO: 9745 - RNA, 20 nt, synthetic construct
  source 1..20: mol_type = other RNA
tgagggccggaaggagctgg

SEQ ID NO: 9746 - RNA, 20 nt, synthetic construct
  source 1..20: mol_type = other RNA
gagggccggaaggagctggg

SEQ ID NO: 9747 - RNA, 20 nt, synthetic construct
  source 1..20: mol_type = other RNA
aggaaccccccagctccttc

SEQ ID NO: 9748 - RNA, 20 nt, synthetic construct
  source 1..20: mol_type = other RNA
gagatgggaagagttagctt

SEQ ID NO: 9749 - RNA, 20 nt, synthetic construct
  source 1..20: mol_type = other RNA
actcttcccatctcccctcc

SEQ ID NO: 9750 - RNA, 20 nt, synthetic construct
  source 1..20: mol_type = other RNA
catctcccctccaggcacgc

SEQ ID NO: 9751 - RNA, 20 nt, synthetic construct
  source 1..20: mol_type = other RNA
tgcgtgcctggaggggagat

SEQ ID NO: 9752 - RNA, 20 nt, synthetic construct
  source 1..20: mol_type = other RNA
ctgcgtgcctggaggggaga

SEQ ID NO: 9753 - RNA, 20 nt, synthetic construct
  source 1..20: mol_type = other RNA
ttcagcctgcgtgcctggag

SEQ ID NO: 9754 - RNA, 20 nt, synthetic construct
  source 1..20: mol_type = other RNA
cttcagcctgcgtgcctgga

SEQ ID NO: 9755 - RNA, 20 nt, synthetic construct
  source 1..20: mol_type = other RNA
tcttcagcctgcgtgcctgg

SEQ ID NO: 9756 - RNA, 20 nt, synthetic construct
  source 1..20: mol_type = other RNA
ctttcttcagcctgcgtgcc

SEQ ID NO: 9757 - RNA, 20 nt, synthetic construct
  source 1..20: mol_type = other RNA
ggctgaagaaagtcccttcg

SEQ ID NO: 9758 - RNA, 20 nt, synthetic construct
  source 1..20: mol_type = other RNA
gctgaagaaagtcccttcgt

SEQ ID NO: 9759 - RNA, 20 nt, synthetic construct
  source 1..20: mol_type = other RNA
agtcccttcgtgggcaaccc

SEQ ID NO: 9760 - RNA, 20 nt, synthetic construct
  source 1..20: mol_type = other RNA
gtcccttcgtgggcaaccca

SEQ ID NO: 9761 - RNA, 20 nt, synthetic construct
  source 1..20: mol_type = other RNA
ttccctgggttgcccacgaa

SEQ ID NO: 9762 - RNA, 20 nt, synthetic construct
  source 1..20: mol_type = other RNA
attccctgggttgcccacga

SEQ ID NO: 9763 - RNA, 20 nt, synthetic construct
  source 1..20: mol_type = other RNA
ggcaacccagggaatatcac

SEQ ID NO: 9764 - RNA, 20 nt, synthetic construct
  source 1..20: mol_type = other RNA
cagggaatatcacaggtgcc

SEQ ID NO: 9765 - RNA, 20 nt, synthetic construct
  source 1..20: mol_type = other RNA
agggaatatcacaggtgccc

SEQ ID NO: 9766 - RNA, 20 nt, synthetic construct
  source 1..20: mol_type = other RNA
gggaatatcacaggtgcccg

SEQ ID NO: 9767 - RNA, 20 nt, synthetic construct
  source 1..20: mol_type = other RNA
gggcacctgtgatattccct

SEQ ID NO: 9768 - RNA, 20 nt, synthetic construct
  source 1..20: mol_type = other RNA
cgggcacctgtgatattccc

SEQ ID NO: 9769 - RNA, 20 nt, synthetic construct
  source 1..20: mol_type = other RNA
cacaggtgcccggggactca

SEQ ID NO: 9770 - RNA, 20 nt, synthetic construct
  source 1..20: mol_type = other RNA
acaggtgcccggggactcac

SEQ ID NO: 9771 - RNA, 20 nt, synthetic construct
  source 1..20: mol_type = other RNA
ggggactcacgggcaccctt

SEQ ID NO: 9772 - RNA, 20 nt, synthetic construct
  source 1..20: mol_type = other RNA
aagggtgcccgtgagtcccc

SEQ ID NO: 9773 - RNA, 20 nt, synthetic construct
  source 1..20: mol_type = other RNA
gaagggtgcccgtgagtccc

SEQ ID NO: 9774 - RNA, 20 nt, synthetic construct
  source 1..20: mol_type = other RNA
cacccttcggtgtcagctcc

SEQ ID NO: 9775 - RNA, 20 nt, synthetic construct
  source 1..20: mol_type = other RNA
tcggtgtcagctccaggttc

SEQ ID NO: 9776 - RNA, 20 nt, synthetic construct
  source 1..20: mol_type = other RNA
cggtgtcagctccaggttca

SEQ ID NO: 9777 - RNA, 20 nt, synthetic construct
  source 1..20: mol_type = other RNA
gaacctggagctgacaccga

SEQ ID NO: 9778 - RNA, 20 nt, synthetic construct
  source 1..20: mol_type = other RNA
ggttcagggagagccccccg

SEQ ID NO: 9779 - RNA, 20 nt, synthetic construct
  source 1..20: mol_type = other RNA
cggggggctctccctgaacc

SEQ ID NO: 9780 - RNA, 20 nt, synthetic construct
  source 1..20: mol_type = other RNA
gagagccccccgaggtacat

SEQ ID NO: 9781 - RNA, 20 nt, synthetic construct
  source 1..20: mol_type = other RNA
cccccgaggtacattggctt

SEQ ID NO: 9782 - RNA, 20 nt, synthetic construct
  source 1..20: mol_type = other RNA
ccccgaggtacattggcttc

SEQ ID NO: 9783 - RNA, 20 nt, synthetic construct
  source 1..20: mol_type = other RNA
cgaagccaatgtacctcggg

SEQ ID NO: 9784 - RNA, 20 nt, synthetic construct
  source 1..20: mol_type = other RNA
gaggtacattggcttcggga

SEQ ID NO: 9785 - RNA, 20 nt, synthetic construct
  source 1..20: mol_type = other RNA
cccgaagccaatgtacctcg

SEQ ID NO: 9786 - RNA, 20 nt, synthetic construct
  source 1..20: mol_type = other RNA
tcccgaagccaatgtacctc

SEQ ID NO: 9787 - RNA, 20 nt, synthetic construct
  source 1..20: mol_type = other RNA
atcccgaagccaatgtacct

SEQ ID NO: 9788 - RNA, 20 nt, synthetic construct
  source 1..20: mol_type = other RNA
gcttcgggatggacagatcc

SEQ ID NO: 9789 - RNA, 20 nt, synthetic construct
  source 1..20: mol_type = other RNA
tggacagatcctggagctcg

SEQ ID NO: 9790 - RNA, 20 nt, synthetic construct
  source 1..20: mol_type = other RNA
gggtgctgtccgcgagctcc

SEQ ID NO: 9791 - RNA, 20 nt, synthetic construct
  source 1..20: mol_type = other RNA
cgcggacagcacccagaccc

SEQ ID NO: 9792 - RNA, 20 nt, synthetic construct
  source 1..20: mol_type = other RNA
cacccagacccaggtgcccc

SEQ ID NO: 9793 - RNA, 20 nt, synthetic construct
  source 1..20: mol_type = other RNA
acccagacccaggtgcccct

SEQ ID NO: 9794 - RNA, 20 nt, synthetic construct
  source 1..20: mol_type = other RNA
gacccaggtgcccctgggtg

SEQ ID NO: 9795 - RNA, 20 nt, synthetic construct
  source 1..20: mol_type = other RNA
acccaggggcacctgggtct

SEQ ID NO: 9796 - RNA, 20 nt, synthetic construct
  source 1..20: mol_type = other RNA
cacccaggggcacctgggtc

SEQ ID NO: 9797 - RNA, 20 nt, synthetic construct
  source 1..20: mol_type = other RNA
atcctcacccaggggcacct

SEQ ID NO: 9798 - RNA, 20 nt, synthetic construct
  source 1..20: mol_type = other RNA
catcctcacccaggggcacc

SEQ ID NO: 9799 - RNA, 20 nt, synthetic construct
  source 1..20: mol_type = other RNA
gcccctgggtgaggatgaac

SEQ ID NO: 9800 - RNA, 20 nt, synthetic construct
  source 1..20: mol_type = other RNA
tcctgttcatcctcacccag

SEQ ID NO: 9801 - RNA, 20 nt, synthetic construct
  source 1..20: mol_type = other RNA
atcctgttcatcctcaccca

SEQ ID NO: 9802 - RNA, 20 nt, synthetic construct
  source 1..20: mol_type = other RNA
gtgaggatgaacaggatgac

SEQ ID NO: 9803 - RNA, 20 nt, synthetic construct
  source 1..20: mol_type = other RNA
tgaacaggatgactggatag

SEQ ID NO: 9804 - RNA, 20 nt, synthetic construct
  source 1..20: mol_type = other RNA
ggatagtggtcagccagctc

SEQ ID NO: 9805 - RNA, 20 nt, synthetic construct
  source 1..20: mol_type = other RNA
ggtcagccagctcaggtgtg

SEQ ID NO: 9806 - RNA, 20 nt, synthetic construct
  source 1..20: mol_type = other RNA
atgtggccacacacctgagc

SEQ ID NO: 9807 - RNA, 20 nt, synthetic construct
  source 1..20: mol_type = other RNA
gggagtgggattcggggatg

SEQ ID NO: 9808 - RNA, 20 nt, synthetic construct
  source 1..20: mol_type = other RNA
ggaggtgggagtgggattcg

SEQ ID NO: 9809 - RNA, 20 nt, synthetic construct
  source 1..20: mol_type = other RNA
cggaggtgggagtgggattc

SEQ ID NO: 9810 - RNA, 20 nt, synthetic construct
  source 1..20: mol_type = other RNA
acggaggtgggagtgggatt

SEQ ID NO: 9811 - RNA, 20 nt, synthetic construct
  source 1..20: mol_type = other RNA
ctcccacctccgtcacacag

SEQ ID NO: 9812 - RNA, 20 nt, synthetic construct
  source 1..20: mol_type = other RNA
tcccacctccgtcacacaga

SEQ ID NO: 9813 - RNA, 20 nt, synthetic construct
  source 1..20: mol_type = other RNA
ctgtgtgacggaggtgggag

SEQ ID NO: 9814 - RNA, 20 nt, synthetic construct
  source 1..20: mol_type = other RNA
gccctctgtgtgacggaggt

SEQ ID NO: 9815 - RNA, 20 nt, synthetic construct
  source 1..20: mol_type = other RNA
tgccctctgtgtgacggagg

SEQ ID NO: 9816 - RNA, 20 nt, synthetic construct
  source 1..20: mol_type = other RNA
ttctgccctctgtgtgacgg

SEQ ID NO: 9817 - RNA, 20 nt, synthetic construct
  source 1..20: mol_type = other RNA
gctttctgccctctgtgtga

SEQ ID NO: 9818 - RNA, 20 nt, synthetic construct
  source 1..20: mol_type = other RNA
cagagggcagaaagcccacc

SEQ ID NO: 9819 - RNA, 20 nt, synthetic construct
  source 1..20: mol_type = other RNA
agagggcagaaagcccacct

SEQ ID NO: 9820 - RNA, 20 nt, synthetic construct
  source 1..20: mol_type = other RNA
gggcagaaagcccacctggg

SEQ ID NO: 9821 - RNA, 20 nt, synthetic construct
  source 1..20: mol_type = other RNA
ggcagaaagcccacctgggt

SEQ ID NO: 9822 - RNA, 20 nt, synthetic construct
  source 1..20: mol_type = other RNA
actggggttcccacccaggt

SEQ ID NO: 9823 - RNA, 20 nt, synthetic construct
  source 1..20: mol_type = other RNA
aactggggttcccacccagg

SEQ ID NO: 9824 - RNA, 20 nt, synthetic construct
  source 1..20: mol_type = other RNA
tcaaactggggttcccaccc

SEQ ID NO: 9825 - RNA, 20 nt, synthetic construct
  source 1..20: mol_type = other RNA
gctgacaagtggtcaaactg

SEQ ID NO: 9826 - RNA, 20 nt, synthetic construct
  source 1..20: mol_type = other RNA
ggctgacaagtggtcaaact

SEQ ID NO: 9827 - RNA, 20 nt, synthetic construct
  source 1..20: mol_type = other RNA
ttgaccacttgtcagccgtg

SEQ ID NO: 9828 - RNA, 20 nt, synthetic construct
  source 1..20: mol_type = other RNA
aaagccgcacggctgacaag

SEQ ID NO: 9829 - RNA, 20 nt, synthetic construct
  source 1..20: mol_type = other RNA
gtgcggctttgagcatgtga

SEQ ID NO: 9830 - RNA, 20 nt, synthetic construct
  source 1..20: mol_type = other RNA
atcacatgctcaaagccgca

SEQ ID NO: 9831 - RNA, 20 nt, synthetic construct
  source 1..20: mol_type = other RNA
gttgtcatgagcttccagac

SEQ ID NO: 9832 - RNA, 20 nt, synthetic construct
  source 1..20: mol_type = other RNA
cggaaagagggtgtccagtc

SEQ ID NO: 9833 - RNA, 20 nt, synthetic construct
  source 1..20: mol_type = other RNA
ggtctgtcagaacggaaaga

SEQ ID NO: 9834 - RNA, 20 nt, synthetic construct
  source 1..20: mol_type = other RNA
gggtctgtcagaacggaaag

SEQ ID NO: 9835 - RNA, 20 nt, synthetic construct
  source 1..20: mol_type = other RNA
tgggagggggtctgtcagaa

SEQ ID NO: 9836 - RNA, 20 nt, synthetic construct
  source 1..20: mol_type = other RNA
cagagctggacactgggagg

SEQ ID NO: 9837 - RNA, 20 nt, synthetic construct
  source 1..20: mol_type = other RNA
tcagagctggacactgggag

SEQ ID NO: 9838 - RNA, 20 nt, synthetic construct
  source 1..20: mol_type = other RNA
gtcagagctggacactggga

SEQ ID NO: 9839 - RNA, 20 nt, synthetic construct
  source 1..20: mol_type = other RNA
ggtcagagctggacactggg

SEQ ID NO: 9840 - RNA, 20 nt, synthetic construct
  source 1..20: mol_type = other RNA
cagggtcagagctggacact

SEQ ID NO: 9841 - RNA, 20 nt, synthetic construct
  source 1..20: mol_type = other RNA
tcagggtcagagctggacac

SEQ ID NO: 9842 - RNA, 20 nt, synthetic construct
  source 1..20: mol_type = other RNA
gagaggttcagggtcagagc

SEQ ID NO: 9843 - RNA, 20 nt, synthetic construct
  source 1..20: mol_type = other RNA
aggagagacagagaggttca

SEQ ID NO: 9844 - RNA, 20 nt, synthetic construct
  source 1..20: mol_type = other RNA
gaggagagacagagaggttc

SEQ ID NO: 9845 - RNA, 20 nt, synthetic construct
  source 1..20: mol_type = other RNA
gggcaagaggagagacagag

SEQ ID NO: 9846 - RNA, 20 nt, synthetic construct
  source 1..20: mol_type = other RNA
ggtgattctgacagggcaag

SEQ ID NO: 9847 - RNA, 20 nt, synthetic construct
  source 1..20: mol_type = other RNA
gcagggaggtgattctgaca

SEQ ID NO: 9848 - RNA, 20 nt, synthetic construct
  source 1..20: mol_type = other RNA
tgcagggaggtgattctgac

SEQ ID NO: 9849 - RNA, 20 nt, synthetic construct
  source 1..20: mol_type = other RNA
ctccctgcagctttccgaca

SEQ ID NO: 9850 - RNA, 20 nt, synthetic construct
  source 1..20: mol_type = other RNA
tccctgcagctttccgacac

SEQ ID NO: 9851 - RNA, 20 nt, synthetic construct
  source 1..20: mol_type = other RNA
cgtgtcggaaagctgcaggg

SEQ ID NO: 9852 - RNA, 20 nt, synthetic construct
  source 1..20: mol_type = other RNA
tcccgtgtcggaaagctgca

SEQ ID NO: 9853 - RNA, 20 nt, synthetic construct
  source 1..20: mol_type = other RNA
gtcccgtgtcggaaagctgc

SEQ ID NO: 9854 - RNA, 20 nt, synthetic construct
  source 1..20: mol_type = other RNA
cacgggacagtaccagtgtt

SEQ ID NO: 9855 - RNA, 20 nt, synthetic construct
  source 1..20: mol_type = other RNA
acactggtactgtcccgtgt

SEQ ID NO: 9856 - RNA, 20 nt, synthetic construct
  source 1..20: mol_type = other RNA
gtaccagtgtttggtgtttc

SEQ ID NO: 9857 - RNA, 20 nt, synthetic construct
  source 1..20: mol_type = other RNA
taccagtgtttggtgtttct

SEQ ID NO: 9858 - RNA, 20 nt, synthetic construct
  source 1..20: mol_type = other RNA
gtcccagaaacaccaaacac

SEQ ID NO: 9859 - RNA, 20 nt, synthetic construct
  source 1..20: mol_type = other RNA
cagaccttcgtgtcccagcc

SEQ ID NO: 9860 - RNA, 20 nt, synthetic construct
  source 1..20: mol_type = other RNA
atagccaggctgggacacga

SEQ ID NO: 9861 - RNA, 20 nt, synthetic construct
  source 1..20: mol_type = other RNA
tgtcccagcctggctatgtt

SEQ ID NO: 9862 - RNA, 20 nt, synthetic construct
  source 1..20: mol_type = other RNA
ccagcctggctatgttgggc

SEQ ID NO: 9863 - RNA, 20 nt, synthetic construct
  source 1..20: mol_type = other RNA
gcctggctatgttgggctgg

SEQ ID NO: 9864 - RNA, 20 nt, synthetic construct
  source 1..20: mol_type = other RNA
cagcccaacatagccaggct

SEQ ID NO: 9865 - RNA, 20 nt, synthetic construct
  source 1..20: mol_type = other RNA
ccagcccaacatagccaggc

SEQ ID NO: 9866 - RNA, 20 nt, synthetic construct
  source 1..20: mol_type = other RNA
ccctccagcccaacatagcc

SEQ ID NO: 9867 - RNA, 20 nt, synthetic construct
  source 1..20: mol_type = other RNA
ttgggctggagggtgagctc

SEQ ID NO: 9868 - RNA, 20 nt, synthetic construct
  source 1..20: mol_type = other RNA
tgggctggagggtgagctct

SEQ ID NO: 9869 - RNA, 20 nt, synthetic construct
  source 1..20: mol_type = other RNA
gggctggagggtgagctctg

SEQ ID NO: 9870 - RNA, 20 nt, synthetic construct
  source 1..20: mol_type = other RNA
ggagggtgagctctggggtc

SEQ ID NO: 9871 - RNA, 20 nt, synthetic construct
  source 1..20: mol_type = other RNA
gagggtgagctctggggtca

SEQ ID NO: 9872 - RNA, 20 nt, synthetic construct
  source 1..20: mol_type = other RNA
agggtgagctctggggtcag

SEQ ID NO: 9873 - RNA, 20 nt, synthetic construct
  source 1..20: mol_type = other RNA
ctctggggtcaggggtcctg

SEQ ID NO: 9874 - RNA, 20 nt, synthetic construct
  source 1..20: mol_type = other RNA
tctggggtcaggggtcctga

SEQ ID NO: 9875 - RNA, 20 nt, synthetic construct
  source 1..20: mol_type = other RNA
ctggggtcaggggtcctgag

SEQ ID NO: 9876 - RNA, 20 nt, synthetic construct
  source 1..20: mol_type = other RNA
caggggtcctgaggggtcag

SEQ ID NO: 9877 - RNA, 20 nt, synthetic construct
  source 1..20: mol_type = other RNA
ctgaggggtcagaggacatg

SEQ ID NO: 9878 - RNA, 20 nt, synthetic construct
  source 1..20: mol_type = other RNA
cacatgtcctctgacccctc

SEQ ID NO: 9879 - RNA, 20 nt, synthetic construct
  source 1..20: mol_type = other RNA
agaggacatgtggcgctcat

SEQ ID NO: 9880 - RNA, 20 nt, synthetic construct
  source 1..20: mol_type = other RNA
catgtggcgctcataggttg

SEQ ID NO: 9881 - RNA, 20 nt, synthetic construct
  source 1..20: mol_type = other RNA
atgtggcgctcataggttgt

SEQ ID NO: 9882 - RNA, 20 nt, synthetic construct
  source 1..20: mol_type = other RNA
ctcataggttgtgggaagtc

SEQ ID NO: 9883 - RNA, 20 nt, synthetic construct
  source 1..20: mol_type = other RNA
gtgggaagtcaggaatcctg

SEQ ID NO: 9884 - RNA, 20 nt, synthetic construct
  source 1..20: mol_type = other RNA
tgggaagtcaggaatcctga

SEQ ID NO: 9885 - RNA, 20 nt, synthetic construct
  source 1..20: mol_type = other RNA
gggaagtcaggaatcctgag

SEQ ID NO: 9886 - RNA, 20 nt, synthetic construct
  source 1..20: mol_type = other RNA
tcaggaatcctgaggggtca

SEQ ID NO: 9887 - RNA, 20 nt, synthetic construct
  source 1..20: mol_type = other RNA
tcctgaggggtcaaggtcaa

SEQ ID NO: 9888 - RNA, 20 nt, synthetic construct
  source 1..20: mol_type = other RNA
cctgaggggtcaaggtcaaa

SEQ ID NO: 9889 - RNA, 20 nt, synthetic construct
  source 1..20: mol_type = other RNA
ccctttgaccttgacccctc

SEQ ID NO: 9890 - RNA, 20 nt, synthetic construct
  source 1..20: mol_type = other RNA
gggtcaaggtcaaagggtgc

SEQ ID NO: 9891 - RNA, 20 nt, synthetic construct
  source 1..20: mol_type = other RNA
tcaaggtcaaagggtgctgg

SEQ ID NO: 9892 - RNA, 20 nt, synthetic construct
  source 1..20: mol_type = other RNA
caaagggtgctggaggattc

SEQ ID NO: 9893 - RNA, 20 nt, synthetic construct
  source 1..20: mol_type = other RNA
aggcaagtcaatgaccctgc

SEQ ID NO: 9894 - RNA, 20 nt, synthetic construct
  source 1..20: mol_type = other RNA
ggcaagtcaatgaccctgca

SEQ ID NO: 9895 - RNA, 20 nt, synthetic construct
  source 1..20: mol_type = other RNA
aagtcaatgaccctgcaggg

SEQ ID NO: 9896 - RNA, 20 nt, synthetic construct
  source 1..20: mol_type = other RNA
agtcaatgaccctgcagggt

SEQ ID NO: 9897 - RNA, 20 nt, synthetic construct
  source 1..20: mol_type = other RNA
ggcagcaaacccaccctgca

SEQ ID NO: 9898 - RNA, 20 nt, synthetic construct
  source 1..20: mol_type = other RNA
gggcagcaaacccaccctgc

SEQ ID NO: 9899 - RNA, 20 nt, synthetic construct
  source 1..20: mol_type = other RNA
caaagcctacagcatcctag

SEQ ID NO: 9900 - RNA, 20 nt, synthetic construct
  source 1..20: mol_type = other RNA
actaggatgctgtaggcttt

SEQ ID NO: 9901 - RNA, 20 nt, synthetic construct
  source 1..20: mol_type = other RNA
cactaggatgctgtaggctt

SEQ ID NO: 9902 - RNA, 20 nt, synthetic construct
  source 1..20: mol_type = other RNA
cagcatcctagtggtgagtc

SEQ ID NO: 9903 - RNA, 20 nt, synthetic construct
  source 1..20: mol_type = other RNA
actcaccactaggatgctgt

SEQ ID NO: 9904 - RNA, 20 nt, synthetic construct
  source 1..20: mol_type = other RNA
tagtggtgagtcaggcatct

SEQ ID NO: 9905 - RNA, 20 nt, synthetic construct
  source 1..20: mol_type = other RNA
agtggtgagtcaggcatctt

SEQ ID NO: 9906 - RNA, 20 nt, synthetic construct
  source 1..20: mol_type = other RNA
gtggtgagtcaggcatcttg

SEQ ID NO: 9907 - RNA, 20 nt, synthetic construct
  source 1..20: mol_type = other RNA
aagatgcctgactcaccact

SEQ ID NO: 9908 - RNA, 20 nt, synthetic construct
  source 1..20: mol_type = other RNA
caggcatcttggggcctcag

SEQ ID NO: 9909 - RNA, 20 nt, synthetic construct
  source 1..20: mol_type = other RNA
aggcatcttggggcctcaga

SEQ ID NO: 9910 - RNA, 20 nt, synthetic construct
  source 1..20: mol_type = other RNA
tagaggctggggtccctctg

SEQ ID NO: 9911 - RNA, 20 nt, synthetic construct
  source 1..20: mol_type = other RNA
gtgggcagtggtagaggctg

SEQ ID NO: 9912 - RNA, 20 nt, synthetic construct
  source 1..20: mol_type = other RNA
ggtgggcagtggtagaggct

SEQ ID NO: 9913 - RNA, 20 nt, synthetic construct
  source 1..20: mol_type = other RNA
gggtgggcagtggtagaggc

SEQ ID NO: 9914 - RNA, 20 nt, synthetic construct
  source 1..20: mol_type = other RNA
ctaccactgcccaccccgct

SEQ ID NO: 9915 - RNA, 20 nt, synthetic construct
  source 1..20: mol_type = other RNA
agcggggtgggcagtggtag

SEQ ID NO: 9916 - RNA, 20 nt, synthetic construct
  source 1..20: mol_type = other RNA
aagcctagcggggtgggcag

SEQ ID NO: 9917 - RNA, 20 nt, synthetic construct
  source 1..20: mol_type = other RNA
taaggcaagcctagcggggt

SEQ ID NO: 9918 - RNA, 20 nt, synthetic construct
  source 1..20: mol_type = other RNA
gtaaggcaagcctagcgggg

SEQ ID NO: 9919 - RNA, 20 nt, synthetic construct
  source 1..20: mol_type = other RNA
gctaggcttgccttacttcc

SEQ ID NO: 9920 - RNA, 20 nt, synthetic construct
  source 1..20: mol_type = other RNA
gaagtaaggcaagcctagcg

SEQ ID NO: 9921 - RNA, 20 nt, synthetic construct
  source 1..20: mol_type = other RNA
ggaagtaaggcaagcctagc

SEQ ID NO: 9922 - RNA, 20 nt, synthetic construct
  source 1..20: mol_type = other RNA
aggaagtaaggcaagcctag

SEQ ID NO: 9923 - RNA, 20 nt, synthetic construct
  source 1..20: mol_type = other RNA
tcgggctcctccaggaagta

SEQ ID NO: 9924 - RNA, 20 nt, synthetic construct
  source 1..20: mol_type = other RNA
tcctggaggagcccgaagac

SEQ ID NO: 9925 - RNA, 20 nt, synthetic construct
  source 1..20: mol_type = other RNA
tcctgtcttcgggctcctcc

SEQ ID NO: 9926 - RNA, 20 nt, synthetic construct
  source 1..20: mol_type = other RNA
ggagcccgaagacaggactg

SEQ ID NO: 9927 - RNA, 20 nt, synthetic construct
  source 1..20: mol_type = other RNA
gcggccacagtcctgtcttc

SEQ ID NO: 9928 - RNA, 20 nt, synthetic construct
  source 1..20: mol_type = other RNA
ggcggccacagtcctgtctt

SEQ ID NO: 9929 - RNA, 20 nt, synthetic construct
  source 1..20: mol_type = other RNA
caggttgaagggggtgttgg

SEQ ID NO: 9930 - RNA, 20 nt, synthetic construct
  source 1..20: mol_type = other RNA
gctcaggttgaagggggtgt

SEQ ID NO: 9931 - RNA, 20 nt, synthetic construct
  source 1..20: mol_type = other RNA
ttggcagctcaggttgaagg

SEQ ID NO: 9932 - RNA, 20 nt, synthetic construct
  source 1..20: mol_type = other RNA
cttggcagctcaggttgaag

SEQ ID NO: 9933 - RNA, 20 nt, synthetic construct
  source 1..20: mol_type = other RNA
caacctgagctgccaagctc

SEQ ID NO: 9934 - RNA, 20 nt, synthetic construct
  source 1..20: mol_type = other RNA
agcttggcagctcaggttga

SEQ ID NO: 9935 - RNA, 20 nt, synthetic construct
  source 1..20: mol_type = other RNA
gtccctgagcttggcagctc

SEQ ID NO: 9936 - RNA, 20 nt, synthetic construct
  source 1..20: mol_type = other RNA
gctctgggggtccctgagct

SEQ ID NO: 9937 - RNA, 20 nt, synthetic construct
  source 1..20: mol_type = other RNA
tcagggacccccagagcccg

SEQ ID NO: 9938 - RNA, 20 nt, synthetic construct
  source 1..20: mol_type = other RNA
cagagcccgtggacctactc

SEQ ID NO: 9939 - RNA, 20 nt, synthetic construct
  source 1..20: mol_type = other RNA
agtaggtccacgggctctgg

SEQ ID NO: 9940 - RNA, 20 nt, synthetic construct
  source 1..20: mol_type = other RNA
gagtaggtccacgggctctg

SEQ ID NO: 9941 - RNA, 20 nt, synthetic construct
  source 1..20: mol_type = other RNA
agagtaggtccacgggctct

SEQ ID NO: 9942 - RNA, 20 nt, synthetic construct
  source 1..20: mol_type = other RNA
cagagtaggtccacgggctc

SEQ ID NO: 9943 - RNA, 20 nt, synthetic construct
  source 1..20: mol_type = other RNA
cgtggacctactctggctcc

SEQ ID NO: 9944 - RNA, 20 nt, synthetic construct
  source 1..20: mol_type = other RNA
tggagccagagtaggtccac

SEQ ID NO: 9945 - RNA, 20 nt, synthetic construct
  source 1..20: mol_type = other RNA
ctggagccagagtaggtcca

SEQ ID NO: 9946 - RNA, 20 nt, synthetic construct
  source 1..20: mol_type = other RNA
cagcatcctggagccagagt

SEQ ID NO: 9947 - RNA, 20 nt, synthetic construct
  source 1..20: mol_type = other RNA
gctccaggatgctgtccccc

SEQ ID NO: 9948 - RNA, 20 nt, synthetic construct
  source 1..20: mol_type = other RNA
ggatgctgtccccctggcca

SEQ ID NO: 9949 - RNA, 20 nt, synthetic construct
  source 1..20: mol_type = other RNA
tggccagggggacagcatcc

SEQ ID NO: 9950 - RNA, 20 nt, synthetic construct
  source 1..20: mol_type = other RNA
gtccccctggccacggctcc

SEQ ID NO: 9951 - RNA, 20 nt, synthetic construct
  source 1..20: mol_type = other RNA
ctggccacggctccaggtca

SEQ ID NO: 9952 - RNA, 20 nt, synthetic construct
  source 1..20: mol_type = other RNA
gacctggagccgtggccagg

SEQ ID NO: 9953 - RNA, 20 nt, synthetic construct
  source 1..20: mol_type = other RNA
tgacctggagccgtggccag

SEQ ID NO: 9954 - RNA, 20 nt, synthetic construct
  source 1..20: mol_type = other RNA
gtgacctggagccgtggcca

SEQ ID NO: 9955 - RNA, 20 nt, synthetic construct
  source 1..20: mol_type = other RNA
cgtgacctggagccgtggcc

SEQ ID NO: 9956 - RNA, 20 nt, synthetic construct
  source 1..20: mol_type = other RNA
ggggccgtgacctggagccg

SEQ ID NO: 9957 - RNA, 20 nt, synthetic construct
  source 1..20: mol_type = other RNA
ctgcgctgggggccgtgacc

SEQ ID NO: 9958 - RNA, 20 nt, synthetic construct
  source 1..20: mol_type = other RNA
cagcgcagcctgcatgttcc

SEQ ID NO: 9959 - RNA, 20 nt, synthetic construct
  source 1..20: mol_type = other RNA
gaacatgcaggctgcgctgg

SEQ ID NO: 9960 - RNA, 20 nt, synthetic construct
  source 1..20: mol_type = other RNA
ggaacatgcaggctgcgctg

SEQ ID NO: 9961 - RNA, 20 nt, synthetic construct
  source 1..20: mol_type = other RNA
tggaacatgcaggctgcgct

SEQ ID NO: 9962 - RNA, 20 nt, synthetic construct
  source 1..20: mol_type = other RNA
ctggaacatgcaggctgcgc

SEQ ID NO: 9963 - RNA, 20 nt, synthetic construct
  source 1..20: mol_type = other RNA
ctgcatgttccaggtgagtc

SEQ ID NO: 9964 - RNA, 20 nt, synthetic construct
  source 1..20: mol_type = other RNA
tgcatgttccaggtgagtcc

SEQ ID NO: 9965 - RNA, 20 nt, synthetic construct
  source 1..20: mol_type = other RNA
gcatgttccaggtgagtccg

SEQ ID NO: 9966 - RNA, 20 nt, synthetic construct
  source 1..20: mol_type = other RNA
cggactcacctggaacatgc

SEQ ID NO: 9967 - RNA, 20 nt, synthetic construct
  source 1..20: mol_type = other RNA
tccaggtgagtccggggatg

SEQ ID NO: 9968 - RNA, 20 nt, synthetic construct
  source 1..20: mol_type = other RNA
ccaggtgagtccggggatgt

SEQ ID NO: 9969 - RNA, 20 nt, synthetic construct
  source 1..20: mol_type = other RNA
cccacatccccggactcacc

SEQ ID NO: 9970 - RNA, 20 nt, synthetic construct
  source 1..20: mol_type = other RNA
tcggagctgacccacatccc

SEQ ID NO: 9971 - RNA, 20 nt, synthetic construct
  source 1..20: mol_type = other RNA
atgtgggtcagctccgaata

SEQ ID NO: 9972 - RNA, 20 nt, synthetic construct
  source 1..20: mol_type = other RNA
tgtgggtcagctccgaatag

SEQ ID NO: 9973 - RNA, 20 nt, synthetic construct
  source 1..20: mol_type = other RNA
gtgggtcagctccgaatagg

SEQ ID NO: 9974 - RNA, 20 nt, synthetic construct
  source 1..20: mol_type = other RNA
gtcagctccgaatagggggc

SEQ ID NO: 9975 - RNA, 20 nt, synthetic construct
  source 1..20: mol_type = other RNA
tcagctccgaatagggggcc

SEQ ID NO: 9976 - RNA, 20 nt, synthetic construct
  source 1..20: mol_type = other RNA
ctccgaatagggggccgggc

SEQ ID NO: 9977 - RNA, 20 nt, synthetic construct
  source 1..20: mol_type = other RNA
tccgaatagggggccgggca

SEQ ID NO: 9978 - RNA, 20 nt, synthetic construct
  source 1..20: mol_type = other RNA
gccctgcccggccccctatt

SEQ ID NO: 9979 - RNA, 20 nt, synthetic construct
  source 1..20: mol_type = other RNA
ggccgggcagggctgaagtc

SEQ ID NO: 9980 - RNA, 20 nt, synthetic construct
  source 1..20: mol_type = other RNA
cagggctgaagtcaggagca

SEQ ID NO: 9981 - RNA, 20 nt, synthetic construct
  source 1..20: mol_type = other RNA
agggctgaagtcaggagcaa

SEQ ID NO: 9982 - RNA, 20 nt, synthetic construct
  source 1..20: mol_type = other RNA
acagtcagacactcacgcag

SEQ ID NO: 9983 - RNA, 20 nt, synthetic construct
  source 1..20: mol_type = other RNA
gacagacagtgagggacaga

SEQ ID NO: 9984 - RNA, 20 nt, synthetic construct
  source 1..20: mol_type = other RNA
ccggtggatcacttgaggtc

SEQ ID NO: 9985 - RNA, 20 nt, synthetic construct
  source 1..20: mol_type = other RNA
ctcaagtgatccaccggcct

SEQ ID NO: 9986 - RNA, 20 nt, synthetic construct
  source 1..20: mol_type = other RNA
cgaggccggtggatcacttg

SEQ ID NO: 9987 - RNA, 20 nt, synthetic construct
  source 1..20: mol_type = other RNA
ctttgggaggccgaggccgg

SEQ ID NO: 9988 - RNA, 20 nt, synthetic construct
  source 1..20: mol_type = other RNA
gcctcggcctcccaaagtac

SEQ ID NO: 9989 - RNA, 20 nt, synthetic construct
  source 1..20: mol_type = other RNA
cctcggcctcccaaagtact

SEQ ID NO: 9990 - RNA, 20 nt, synthetic construct
  source 1..20: mol_type = other RNA
gtactttgggaggccgaggc

SEQ ID NO: 9991 - RNA, 20 nt, synthetic construct
  source 1..20: mol_type = other RNA
cccagtactttgggaggccg

SEQ ID NO: 9992 - RNA, 20 nt, synthetic construct
  source 1..20: mol_type = other RNA
tcccaaagtactgggattac

SEQ ID NO: 9993 - RNA, 20 nt, synthetic construct
  source 1..20: mol_type = other RNA
tgtaatcccagtactttggg

SEQ ID NO: 9994 - RNA, 20 nt, synthetic construct
  source 1..20: mol_type = other RNA
gcctgtaatcccagtacttt

SEQ ID NO: 9995 - RNA, 20 nt, synthetic construct
  source 1..20: mol_type = other RNA
cgcctgtaatcccagtactt

SEQ ID NO: 9996 - RNA, 20 nt, synthetic construct
  source 1..20: mol_type = other RNA
cacatttgcgctgggtgcgg

SEQ ID NO: 9997 - RNA, 20 nt, synthetic construct
  source 1..20: mol_type = other RNA
aaacacatttgcgctgggtg

SEQ ID NO: 9998 - RNA, 20 nt, synthetic construct
  source 1..20: mol_type = other RNA
tacaaaaacacatttgcgct

SEQ ID NO: 9999 - RNA, 20 nt, synthetic construct
  source 1..20: mol_type = other RNA
atacaaaaacacatttgcgc

SEQ ID NO: 10000 - RNA, 20 nt, synthetic construct
  source 1..20: mol_type = other RNA
tttttgtatcagtctgtgtc

SEQ ID NO: 10001 - RNA, 20 nt, synthetic construct
  source 1..20: mol_type = other RNA
ttttgtatcagtctgtgtct

SEQ ID NO: 10002 - RNA, 20 nt, synthetic construct
  source 1..20: mol_type = other RNA
gtctgggtgaacatgaaacc

SEQ ID NO: 10003 - RNA, 20 nt, synthetic construct
  source 1..20: mol_type = other RNA
tctgggtgaacatgaaacct

SEQ ID NO: 10004 - RNA, 20 nt, synthetic construct
  source 1..20: mol_type = other RNA
agatggagctggatgcgccc

SEQ ID NO: 10005 - RNA, 20 nt, synthetic construct
  source 1..20: mol_type = other RNA
gctccatcttatggcgtaga

SEQ ID NO: 10006 - RNA, 20 nt, synthetic construct
  source 1..20: mol_type = other RNA
tctacgccataagatggagc

SEQ ID NO: 10007 - RNA, 20 nt, synthetic construct
  source 1..20: mol_type = other RNA
ccatcttatggcgtagatgg

SEQ ID NO: 10008 - RNA, 20 nt, synthetic construct
  source 1..20: mol_type = other RNA
ttatggcgtagatggaggct

SEQ ID NO: 10009 - RNA, 20 nt, synthetic construct
  source 1..20: mol_type = other RNA
tagatggaggcttggctgtg

SEQ ID NO: 10010 - RNA, 20 nt, synthetic construct
  source 1..20: mol_type = other RNA
tggctgtgaggtgtacgcgt

SEQ ID NO: 10011 - RNA, 20 nt, synthetic construct
  source 1..20: mol_type = other RNA
cggtgtgtctgtgtctgagc

SEQ ID NO: 10012 - RNA, 20 nt, synthetic construct
  source 1..20: mol_type = other RNA
aatgacccttcattgtgtcc

SEQ ID NO: 10013 - RNA, 20 nt, synthetic construct
  source 1..20: mol_type = other RNA
acacaccaggacacaatgaa

SEQ ID NO: 10014 - RNA, 20 nt, synthetic construct
  source 1..20: mol_type = other RNA
tacacaccaggacacaatga

SEQ ID NO: 10015 - RNA, 20 nt, synthetic construct
  source 1..20: mol_type = other RNA
tggacagatagatacacacc

SEQ ID NO: 10016 - RNA, 20 nt, synthetic construct
  source 1..20: mol_type = other RNA
cagcgtacatggagttgagg

SEQ ID NO: 10017 - RNA, 20 nt, synthetic construct
  source 1..20: mol_type = other RNA
taacagcgtacatggagttg

SEQ ID NO: 10018 - RNA, 20 nt, synthetic construct
  source 1..20: mol_type = other RNA
acaccacgtaacagcgtaca

SEQ ID NO: 10019 - RNA, 20 nt, synthetic construct
  source 1..20: mol_type = other RNA
gtgtgtgtctctgaatatac

SEQ ID NO: 10020 - RNA, 20 nt, synthetic construct
  source 1..20: mol_type = other RNA
tgtgtgtctctgaatataca

SEQ ID NO: 10021 - RNA, 20 nt, synthetic construct
  source 1..20: mol_type = other RNA
atttaagtttctgtgtgtgt

SEQ ID NO: 10022 - RNA, 20 nt, synthetic construct
  source 1..20: mol_type = other RNA
tagatgtacattgcgtcgct

SEQ ID NO: 10023 - RNA, 20 nt, synthetic construct
  source 1..20: mol_type = other RNA
tagcgacgcaatgtacatct

SEQ ID NO: 10024 - RNA, 20 nt, synthetic construct
  source 1..20: mol_type = other RNA
tttatgtgtttgtcccacgt

SEQ ID NO: 10025 - RNA, 20 nt, synthetic construct
  source 1..20: mol_type = other RNA
gtatgcatacaagccaacgt

SEQ ID NO: 10026 - RNA, 20 nt, synthetic construct
  source 1..20: mol_type = other RNA
tgtatgcatacaagccaacg

SEQ ID NO: 10027 - RNA, 20 nt, synthetic construct
  source 1..20: mol_type = other RNA
gcgtgtatatgtgtgagtca

SEQ ID NO: 10028 - RNA, 20 nt, synthetic construct
  source 1..20: mol_type = other RNA
tgactcacacatatacacgc

SEQ ID NO: 10029 - RNA, 20 nt, synthetic construct
  source 1..20: mol_type = other RNA
gtgactcacacatatacacg

SEQ ID NO: 10030 - RNA, 20 nt, synthetic construct
  source 1..20: mol_type = other RNA
aacggcacacagatatgcaa

SEQ ID NO: 10031 - RNA, 20 nt, synthetic construct
  source 1..20: mol_type = other RNA
taacggcacacagatatgca

SEQ ID NO: 10032 - RNA, 20 nt, synthetic construct
  source 1..20: mol_type = other RNA
cgcagcgcttggtaagttaa

SEQ ID NO: 10033 - RNA, 20 nt, synthetic construct
  source 1..20: mol_type = other RNA
agcacagaagacgcagcgct

SEQ ID NO: 10034 - RNA, 20 nt, synthetic construct
  source 1..20: mol_type = other RNA
aatcacacttaaacacacag

SEQ ID NO: 10035 - RNA, 20 nt, synthetic construct
  source 1..20: mol_type = other RNA
gaatcacacttaaacacaca

SEQ ID NO: 10036 - RNA, 20 nt, synthetic construct
  source 1..20: mol_type = other RNA
tgaatcacacttaaacacac

SEQ ID NO: 10037 - RNA, 20 nt, synthetic construct
  source 1..20: mol_type = other RNA
attcattgtgagtgtgtgtg

SEQ ID NO: 10038 - RNA, 20 nt, synthetic construct
  source 1..20: mol_type = other RNA
ttcattgtgagtgtgtgtgt

SEQ ID NO: 10039 - RNA, 20 nt, synthetic construct
  source 1..20: mol_type = other RNA
tcattgtgagtgtgtgtgtg

SEQ ID NO: 10040 - RNA, 20 nt, synthetic construct
  source 1..20: mol_type = other RNA
cattgtgagtgtgtgtgtgg

SEQ ID NO: 10041 - RNA, 20 nt, synthetic construct
  source 1..20: mol_type = other RNA
attgtgagtgtgtgtgtggg

SEQ ID NO: 10042 - RNA, 20 nt, synthetic construct
  source 1..20: mol_type = other RNA
ttgtgagtgtgtgtgtgggg

SEQ ID NO: 10043 - RNA, 20 nt, synthetic construct
  source 1..20: mol_type = other RNA
tgggggggtttgctgtgtga

SEQ ID NO: 10044 - RNA, 20 nt, synthetic construct
  source 1..20: mol_type = other RNA
gagggacagacgcacacaaa

SEQ ID NO: 10045 - RNA, 20 nt, synthetic construct
  source 1..20: mol_type = other RNA
tctgtccctctatctgactc

SEQ ID NO: 10046 - RNA, 20 nt, synthetic construct
  source 1..20: mol_type = other RNA
ctgtccctctatctgactca

SEQ ID NO: 10047 - RNA, 20 nt, synthetic construct
  source 1..20: mol_type = other RNA
cacgccctgagtcagataga

SEQ ID NO: 10048 - RNA, 20 nt, synthetic construct
  source 1..20: mol_type = other RNA
gcacgccctgagtcagatag

SEQ ID NO: 10049 - RNA, 20 nt, synthetic construct
  source 1..20: mol_type = other RNA
gagagggatggaaggaggag

SEQ ID NO: 10050 - RNA, 20 nt, synthetic construct
  source 1..20: mol_type = other RNA
tgagagggatggaaggagga

SEQ ID NO: 10051 - RNA, 20 nt, synthetic construct
  source 1..20: mol_type = other RNA
atgagagggatggaaggagg

SEQ ID NO: 10052 - RNA, 20 nt, synthetic construct
  source 1..20: mol_type = other RNA
cttccatccctctcattctc

SEQ ID NO: 10053 - RNA, 20 nt, synthetic construct
  source 1..20: mol_type = other RNA
agaatgagagggatggaagg

SEQ ID NO: 10054 - RNA, 20 nt, synthetic construct
  source 1..20: mol_type = other RNA
cagagaatgagagggatgga

SEQ ID NO: 10055 - RNA, 20 nt, synthetic construct
  source 1..20: mol_type = other RNA
tttccagagaatgagaggga

SEQ ID NO: 10056 - RNA, 20 nt, synthetic construct
  source 1..20: mol_type = other RNA
ctctcattctctggaaaagc

SEQ ID NO: 10057 - RNA, 20 nt, synthetic construct
  source 1..20: mol_type = other RNA
tctcattctctggaaaagct

SEQ ID NO: 10058 - RNA, 20 nt, synthetic construct
  source 1..20: mol_type = other RNA
ctcattctctggaaaagctg

SEQ ID NO: 10059 - RNA, 20 nt, synthetic construct
  source 1..20: mol_type = other RNA
agcttttccagagaatgaga

SEQ ID NO: 10060 - RNA, 20 nt, synthetic construct
  source 1..20: mol_type = other RNA
cagcttttccagagaatgag

SEQ ID NO: 10061 - RNA, 20 nt, synthetic construct
  source 1..20: mol_type = other RNA
attctctggaaaagctgggg

SEQ ID NO: 10062 - RNA, 20 nt, synthetic construct
  source 1..20: mol_type = other RNA
gaaaagctggggcggagagc

SEQ ID NO: 10063 - RNA, 20 nt, synthetic construct
  source 1..20: mol_type = other RNA
aaaagctggggcggagagca

SEQ ID NO: 10064 - RNA, 20 nt, synthetic construct
  source 1..20: mol_type = other RNA
aaagctggggcggagagcag

SEQ ID NO: 10065 - RNA, 20 nt, synthetic construct
  source 1..20: mol_type = other RNA
ggggcggagagcaggggttg

SEQ ID NO: 10066 - RNA, 20 nt, synthetic construct
  source 1..20: mol_type = other RNA
gggcggagagcaggggttgt

SEQ ID NO: 10067 - RNA, 20 nt, synthetic construct
  source 1..20: mol_type = other RNA
ggcggagagcaggggttgtg

SEQ ID NO: 10068 - RNA, 20 nt, synthetic construct
  source 1..20: mol_type = other RNA
gcggagagcaggggttgtgg

SEQ ID NO: 10069 - RNA, 20 nt, synthetic construct
  source 1..20: mol_type = other RNA
cggagagcaggggttgtggg

SEQ ID NO: 10070 - RNA, 20 nt, synthetic construct
  source 1..20: mol_type = other RNA
gagcaggggttgtgggggga

SEQ ID NO: 10071 - RNA, 20 nt, synthetic construct
  source 1..20: mol_type = other RNA
ggggttgtggggggatggtc

SEQ ID NO: 10072 - RNA, 20 nt, synthetic construct
  source 1..20: mol_type = other RNA
ggggggatggtcaggacatc

SEQ ID NO: 10073 - RNA, 20 nt, synthetic construct
  source 1..20: mol_type = other RNA
ggacatctggaaagcacatc

SEQ ID NO: 10074 - RNA, 20 nt, synthetic construct
  source 1..20: mol_type = other RNA
ctggaaagcacatctggaat

SEQ ID NO: 10075 - RNA, 20 nt, synthetic construct
  source 1..20: mol_type = other RNA
ggcctgctcctgtcgtcttg

SEQ ID NO: 10076 - RNA, 20 nt, synthetic construct
  source 1..20: mol_type = other RNA
taccgcaagacgacaggagc

SEQ ID NO: 10077 - RNA, 20 nt, synthetic construct
  source 1..20: mol_type = other RNA
ttgctttaccgcaagacgac

SEQ ID NO: 10078 - RNA, 20 nt, synthetic construct
  source 1..20: mol_type = other RNA
gcggtaaagcaagaaccttc

SEQ ID NO: 10079 - RNA, 20 nt, synthetic construct
  source 1..20: mol_type = other RNA
gtaaagcaagaaccttctgg

SEQ ID NO: 10080 - RNA, 20 nt, synthetic construct
  source 1..20: mol_type = other RNA
taaagcaagaaccttctgga

SEQ ID NO: 10081 - RNA, 20 nt, synthetic construct
  source 1..20: mol_type = other RNA
aaagcaagaaccttctggag

SEQ ID NO: 10082 - RNA, 20 nt, synthetic construct
  source 1..20: mol_type = other RNA
caagaaccttctggagggga

SEQ ID NO: 10083 - RNA, 20 nt, synthetic construct
  source 1..20: mol_type = other RNA
aagaaccttctggaggggaa

SEQ ID NO: 10084 - RNA, 20 nt, synthetic construct
  source 1..20: mol_type = other RNA
agaaccttctggaggggaag

SEQ ID NO: 10085 - RNA, 20 nt, synthetic construct
  source 1..20: mol_type = other RNA
gggaccccttcccctccaga

SEQ ID NO: 10086 - RNA, 20 nt, synthetic construct
  source 1..20: mol_type = other RNA
tgaaggggacaggaggaact

SEQ ID NO: 10087 - RNA, 20 nt, synthetic construct
  source 1..20: mol_type = other RNA
gtgaaggggacaggaggaac

SEQ ID NO: 10088 - RNA, 20 nt, synthetic construct
  source 1..20: mol_type = other RNA
cctcctgtccccttcactca

SEQ ID NO: 10089 - RNA, 20 nt, synthetic construct
  source 1..20: mol_type = other RNA
tgtccccttcactcaaggtg

SEQ ID NO: 10090 - RNA, 20 nt, synthetic construct
  source 1..20: mol_type = other RNA
gcaccttgagtgaaggggac

SEQ ID NO: 10091 - RNA, 20 nt, synthetic construct
  source 1..20: mol_type = other RNA
ttcactcaaggtgcggccgt

SEQ ID NO: 10092 - RNA, 20 nt, synthetic construct
  source 1..20: mol_type = other RNA
tcactcaaggtgcggccgtt

SEQ ID NO: 10093 - RNA, 20 nt, synthetic construct
  source 1..20: mol_type = other RNA
acggccgcaccttgagtgaa

SEQ ID NO: 10094 - RNA, 20 nt, synthetic construct
  source 1..20: mol_type = other RNA
aacggccgcaccttgagtga

SEQ ID NO: 10095 - RNA, 20 nt, synthetic construct
  source 1..20: mol_type = other RNA
aaggtgcggccgttggggcc

SEQ ID NO: 10096 - RNA, 20 nt, synthetic construct
  source 1..20: mol_type = other RNA
aggtgcggccgttggggcct

SEQ ID NO: 10097 - RNA, 20 nt, synthetic construct
  source 1..20: mol_type = other RNA
gcggccgttggggcctggga

SEQ ID NO: 10098 - RNA, 20 nt, synthetic construct
  source 1..20: mol_type = other RNA
cggccgttggggcctgggaa

SEQ ID NO: 10099 - RNA, 20 nt, synthetic construct
  source 1..20: mol_type = other RNA
ggccgttggggcctgggaag

SEQ ID NO: 10100 - RNA, 20 nt, synthetic construct
  source 1..20: mol_type = other RNA
gccgttggggcctgggaagg

SEQ ID NO: 10101 - RNA, 20 nt, synthetic construct
  source 1..20: mol_type = other RNA
tcccccttcccaggccccaa

SEQ ID NO: 10102 - RNA, 20 nt, synthetic construct
  source 1..20: mol_type = other RNA
gggcctgggaagggggatcc

SEQ ID NO: 10103 - RNA, 20 nt, synthetic construct
  source 1..20: mol_type = other RNA
gggaagggggatcccggctc

SEQ ID NO: 10104 - RNA, 20 nt, synthetic construct
  source 1..20: mol_type = other RNA
gagccgggatcccccttccc

SEQ ID NO: 10105 - RNA, 20 nt, synthetic construct
  source 1..20: mol_type = other RNA
gggggcgcggagccagagcc

SEQ ID NO: 10106 - RNA, 20 nt, synthetic construct
  source 1..20: mol_type = other RNA
cgggggcgcggagccagagc

SEQ ID NO: 10107 - RNA, 20 nt, synthetic construct
  source 1..20: mol_type = other RNA
tggctccgcgcccccgaagc

SEQ ID NO: 10108 - RNA, 20 nt, synthetic construct
  source 1..20: mol_type = other RNA
tccgcgcccccgaagccggc

SEQ ID NO: 10109 - RNA, 20 nt, synthetic construct
  source 1..20: mol_type = other RNA
tccggccggcttcgggggcg

SEQ ID NO: 10110 - RNA, 20 nt, synthetic construct
  source 1..20: mol_type = other RNA
ccgaagccggccggaagcgc

SEQ ID NO: 10111 - RNA, 20 nt, synthetic construct
  source 1..20: mol_type = other RNA
cgaagccggccggaagcgct

SEQ ID NO: 10112 - RNA, 20 nt, synthetic construct
  source 1..20: mol_type = other RNA
gcgcttccggccggcttcgg

SEQ ID NO: 10113 - RNA, 20 nt, synthetic construct
  source 1..20: mol_type = other RNA
agcgcttccggccggcttcg

SEQ ID NO: 10114 - RNA, 20 nt, synthetic construct
  source 1..20: mol_type = other RNA
cagcgcttccggccggcttc

SEQ ID NO: 10115 - RNA, 20 nt, synthetic construct
  source 1..20: mol_type = other RNA
ccagcgcttccggccggctt

SEQ ID NO: 10116 - RNA, 20 nt, synthetic construct
  source 1..20: mol_type = other RNA
ccggccggaagcgctggggt

SEQ ID NO: 10117 - RNA, 20 nt, synthetic construct
  source 1..20: mol_type = other RNA
cggccggaagcgctggggtg

SEQ ID NO: 10118 - RNA, 20 nt, synthetic construct
  source 1..20: mol_type = other RNA
ccggaagcgctggggtgggg

SEQ ID NO: 10119 - RNA, 20 nt, synthetic construct
  source 1..20: mol_type = other RNA
cccaccccagcgcttccggc

SEQ ID NO: 10120 - RNA, 20 nt, synthetic construct
  source 1..20: mol_type = other RNA
cctccccaccccagcgcttc

SEQ ID NO: 10121 - RNA, 20 nt, synthetic construct
  source 1..20: mol_type = other RNA
ctggggtggggaggtgcccc

SEQ ID NO: 10122 - RNA, 20 nt, synthetic construct
  source 1..20: mol_type = other RNA
ggtgcccccggtgactcacg

SEQ ID NO: 10123 - RNA, 20 nt, synthetic construct
  source 1..20: mol_type = other RNA
gtgcccccggtgactcacgc

SEQ ID NO: 10124 - RNA, 20 nt, synthetic construct
  source 1..20: mol_type = other RNA
tgcccccggtgactcacgcg

SEQ ID NO: 10125 - RNA, 20 nt, synthetic construct
  source 1..20: mol_type = other RNA
gcccccggtgactcacgcgg

SEQ ID NO: 10126 - RNA, 20 nt, synthetic construct
  source 1..20: mol_type = other RNA
ccggtgactcacgcgggggc

SEQ ID NO: 10127 - RNA, 20 nt, synthetic construct
  source 1..20: mol_type = other RNA
gcccccgcgtgagtcaccgg

SEQ ID NO: 10128 - RNA, 20 nt, synthetic construct
  source 1..20: mol_type = other RNA
tgcccccgcgtgagtcaccg

SEQ ID NO: 10129 - RNA, 20 nt, synthetic construct
  source 1..20: mol_type = other RNA
ctgcccccgcgtgagtcacc

SEQ ID NO: 10130 - RNA, 20 nt, synthetic construct
  source 1..20: mol_type = other RNA
cctgcccccgcgtgagtcac

SEQ ID NO: 10131 - RNA, 20 nt, synthetic construct
  source 1..20: mol_type = other RNA
acgcgggggcaggaatgctg

SEQ ID NO: 10132 - RNA, 20 nt, synthetic construct
  source 1..20: mol_type = other RNA
gggggcaggaatgctgcggt

SEQ ID NO: 10133 - RNA, 20 nt, synthetic construct
  source 1..20: mol_type = other RNA
caggaatgctgcggtcggaa

SEQ ID NO: 10134 - RNA, 20 nt, synthetic construct
  source 1..20: mol_type = other RNA
aggaatgctgcggtcggaac

SEQ ID NO: 10135 - RNA, 20 nt, synthetic construct
  source 1..20: mol_type = other RNA
gctgcggtcggaacgggacc

SEQ ID NO: 10136 - RNA, 20 nt, synthetic construct
  source 1..20: mol_type = other RNA
tggaggtgggttctggagcc

SEQ ID NO: 10137 - RNA, 20 nt, synthetic construct
  source 1..20: mol_type = other RNA
ctggaggtgggttctggagc

SEQ ID NO: 10138 - RNA, 20 nt, synthetic construct
  source 1..20: mol_type = other RNA
cagaacccacctccagcccc

SEQ ID NO: 10139 - RNA, 20 nt, synthetic construct
  source 1..20: mol_type = other RNA
agaacccacctccagcccca

SEQ ID NO: 10140 - RNA, 20 nt, synthetic construct
  source 1..20: mol_type = other RNA
ctggggctggaggtgggttc

SEQ ID NO: 10141 - RNA, 20 nt, synthetic construct
  source 1..20: mol_type = other RNA
gaagccctggggctggaggt

SEQ ID NO: 10142 - RNA, 20 nt, synthetic construct
  source 1..20: mol_type = other RNA
agaagccctggggctggagg

SEQ ID NO: 10143 - RNA, 20 nt, synthetic construct
  source 1..20: mol_type = other RNA
cggagaagccctggggctgg

SEQ ID NO: 10144 - RNA, 20 nt, synthetic construct
  source 1..20: mol_type = other RNA
cccagggcttctccggccgg

SEQ ID NO: 10145 - RNA, 20 nt, synthetic construct
  source 1..20: mol_type = other RNA
cgccggccggagaagccctg

SEQ ID NO: 10146 - RNA, 20 nt, synthetic construct
  source 1..20: mol_type = other RNA
ccgccggccggagaagccct

SEQ ID NO: 10147 - RNA, 20 nt, synthetic construct
  source 1..20: mol_type = other RNA
gccgccggccggagaagccc

SEQ ID NO: 10148 - RNA, 20 nt, synthetic construct
  source 1..20: mol_type = other RNA
cgggagctggcgccgccggc

SEQ ID NO: 10149 - RNA, 20 nt, synthetic construct
  source 1..20: mol_type = other RNA
cgcgcgggagctggcgccgc

SEQ ID NO: 10150 - RNA, 20 nt, synthetic construct
  source 1..20: mol_type = other RNA
cagctcccgcgcgctgaccc

SEQ ID NO: 10151 - RNA, 20 nt, synthetic construct
  source 1..20: mol_type = other RNA
ctcccgcgcgctgaccctgg

SEQ ID NO: 10152 - RNA, 20 nt, synthetic construct
  source 1..20: mol_type = other RNA
tcccgcgcgctgaccctggc

SEQ ID NO: 10153 - RNA, 20 nt, synthetic construct
  source 1..20: mol_type = other RNA
cccgcgcgctgaccctggcg

SEQ ID NO: 10154 - RNA, 20 nt, synthetic construct
  source 1..20: mol_type = other RNA
ccccgccagggtcagcgcgc

SEQ ID NO: 10155 - RNA, 20 nt, synthetic construct
  source 1..20: mol_type = other RNA
gccccgccagggtcagcgcg

SEQ ID NO: 10156 - RNA, 20 nt, synthetic construct
  source 1..20: mol_type = other RNA
ctggcggggccccacgtgcc

SEQ ID NO: 10157 - RNA, 20 nt, synthetic construct
  source 1..20: mol_type = other RNA
gcggggccccacgtgccagg

SEQ ID NO: 10158 - RNA, 20 nt, synthetic construct
  source 1..20: mol_type = other RNA
ctggcacgtggggccccgcc

SEQ ID NO: 10159 - RNA, 20 nt, synthetic construct
  source 1..20: mol_type = other RNA
ggccccacgtgccaggtggc

SEQ ID NO: 10160 - RNA, 20 nt, synthetic construct
  source 1..20: mol_type = other RNA
gtccagccacctggcacgtg

SEQ ID NO: 10161 - RNA, 20 nt, synthetic construct
  source 1..20: mol_type = other RNA
ggtccagccacctggcacgt

SEQ ID NO: 10162 - RNA, 20 nt, synthetic construct
  source 1..20: mol_type = other RNA
gggtccagccacctggcacg

SEQ ID NO: 10163 - RNA, 20 nt, synthetic construct
  source 1..20: mol_type = other RNA
caggtggctggacccgaccc

SEQ ID NO: 10164 - RNA, 20 nt, synthetic construct
  source 1..20: mol_type = other RNA
ctgggtcgggtccagccacc

SEQ ID NO: 10165 - RNA, 20 nt, synthetic construct
  source 1..20: mol_type = other RNA
gggggcggggagcctgggtc

SEQ ID NO: 10166 - RNA, 20 nt, synthetic construct
  source 1..20: mol_type = other RNA
ccaggctccccgcccccact

SEQ ID NO: 10167 - RNA, 20 nt, synthetic construct
  source 1..20: mol_type = other RNA
caggctccccgcccccactc

SEQ ID NO: 10168 - RNA, 20 nt, synthetic construct
  source 1..20: mol_type = other RNA
cgagtgggggcggggagcct

SEQ ID NO: 10169 - RNA, 20 nt, synthetic construct
  source 1..20: mol_type = other RNA
ccgagtgggggcggggagcc

SEQ ID NO: 10170 - RNA, 20 nt, synthetic construct
  source 1..20: mol_type = other RNA
gggcggcccgagtgggggcg

SEQ ID NO: 10171 - RNA, 20 nt, synthetic construct
  source 1..20: mol_type = other RNA
cgggcggcccgagtgggggc

SEQ ID NO: 10172 - RNA, 20 nt, synthetic construct
  source 1..20: mol_type = other RNA
gcgggcggcccgagtggggg

SEQ ID NO: 10173 - RNA, 20 nt, synthetic construct
  source 1..20: mol_type = other RNA
cgggcgggcggcccgagtgg

SEQ ID NO: 10174 - RNA, 20 nt, synthetic construct
  source 1..20: mol_type = other RNA
ccgggcgggcggcccgagtg

SEQ ID NO: 10175 - RNA, 20 nt, synthetic construct
  source 1..20: mol_type = other RNA
cccgggcgggcggcccgagt

SEQ ID NO: 10176 - RNA, 20 nt, synthetic construct
  source 1..20: mol_type = other RNA
tcccgggcgggcggcccgag

SEQ ID NO: 10177 - RNA, 20 nt, synthetic construct
  source 1..20: mol_type = other RNA
acagtacagtcccgggcggg

SEQ ID NO: 10178 - RNA, 20 nt, synthetic construct
  source 1..20: mol_type = other RNA
gaaacagtacagtcccgggc

SEQ ID NO: 10179 - RNA, 20 nt, synthetic construct
  source 1..20: mol_type = other RNA
agaaacagtacagtcccggg

SEQ ID NO: 10180 - RNA, 20 nt, synthetic construct
  source 1..20: mol_type = other RNA
ggactgtactgtttctcctc

SEQ ID NO: 10181 - RNA, 20 nt, synthetic construct
  source 1..20: mol_type = other RNA
gactgtactgtttctcctcc

SEQ ID NO: 10182 - RNA, 20 nt, synthetic construct
  source 1..20: mol_type = other RNA
gaggagaaacagtacagtcc

SEQ ID NO: 10183 - RNA, 20 nt, synthetic construct
  source 1..20: mol_type = other RNA
tgtactgtttctcctccggg

SEQ ID NO: 10184 - RNA, 20 nt, synthetic construct
  source 1..20: mol_type = other RNA
tgtttctcctccgggcggcg

SEQ ID NO: 10185 - RNA, 20 nt, synthetic construct
  source 1..20: mol_type = other RNA
gtttctcctccgggcggcgc

SEQ ID NO: 10186 - RNA, 20 nt, synthetic construct
  source 1..20: mol_type = other RNA
tttctcctccgggcggcgcg

SEQ ID NO: 10187 - RNA, 20 nt, synthetic construct
  source 1..20: mol_type = other RNA
ttctcctccgggcggcgcgg

SEQ ID NO: 10188 - RNA, 20 nt, synthetic construct
  source 1..20: mol_type = other RNA
tccgggcggcgcgggggctg

SEQ ID NO: 10189 - RNA, 20 nt, synthetic construct
  source 1..20: mol_type = other RNA
ccgggcggcgcgggggctgc

SEQ ID NO: 10190 - RNA, 20 nt, synthetic construct
  source 1..20: mol_type = other RNA
gcagcccccgcgccgcccgg

SEQ ID NO: 10191 - RNA, 20 nt, synthetic construct
  source 1..20: mol_type = other RNA
cggcgcgggggctgcgggcg

SEQ ID NO: 10192 - RNA, 20 nt, synthetic construct
  source 1..20: mol_type = other RNA
ggcgcgggggctgcgggcgc

SEQ ID NO: 10193 - RNA, 20 nt, synthetic construct
  source 1..20: mol_type = other RNA
gcgcgggggctgcgggcgcg

SEQ ID NO: 10194 - RNA, 20 nt, synthetic construct
  source 1..20: mol_type = other RNA
gctgcgggcgcggggccttc

SEQ ID NO: 10195 - RNA, 20 nt, synthetic construct
  source 1..20: mol_type = other RNA
ctgcgggcgcggggccttca

SEQ ID NO: 10196 - RNA, 20 nt, synthetic construct
  source 1..20: mol_type = other RNA
ggcgcggggccttcagggcg

SEQ ID NO: 10197 - RNA, 20 nt, synthetic construct
  source 1..20: mol_type = other RNA
gcggggccttcagggcgcgg

SEQ ID NO: 10198 - RNA, 20 nt, synthetic construct
  source 1..20: mol_type = other RNA
ccttcagggcgcggaggctg

SEQ ID NO: 10199 - RNA, 20 nt, synthetic construct
  source 1..20: mol_type = other RNA
cttcagggcgcggaggctgc

SEQ ID NO: 10200 - RNA, 20 nt, synthetic construct
  source 1..20: mol_type = other RNA
ccgcagcctccgcgccctga

SEQ ID NO: 10201 - RNA, 20 nt, synthetic construct
  source 1..20: mol_type = other RNA
gggcgcggaggctgcgggag

SEQ ID NO: 10202 - RNA, 20 nt, synthetic construct
  source 1..20: mol_type = other RNA
ggcgcggaggctgcgggagc

SEQ ID NO: 10203 - RNA, 20 nt, synthetic construct
  source 1..20: mol_type = other RNA
agcgggcacctgaccttgtc

SEQ ID NO: 10204 - RNA, 20 nt, synthetic construct
  source 1..20: mol_type = other RNA
gcgggcacctgaccttgtct

SEQ ID NO: 10205 - RNA, 20 nt, synthetic construct
  source 1..20: mol_type = other RNA
cacctgaccttgtctgggaa

SEQ ID NO: 10206 - RNA, 20 nt, synthetic construct
  source 1..20: mol_type = other RNA
ggccgttcccagacaaggtc

SEQ ID NO: 10207 - RNA, 20 nt, synthetic construct
  source 1..20: mol_type = other RNA
ttgtctgggaacggccacct

SEQ ID NO: 10208 - RNA, 20 nt, synthetic construct
  source 1..20: mol_type = other RNA
taggtggccgttcccagaca

SEQ ID NO: 10209 - RNA, 20 nt, synthetic construct
  source 1..20: mol_type = other RNA
cacctaggaagccgcgactg

SEQ ID NO: 10210 - RNA, 20 nt, synthetic construct
  source 1..20: mol_type = other RNA
ctcagtcgcggcttcctagg

SEQ ID NO: 10211 - RNA, 20 nt, synthetic construct
  source 1..20: mol_type = other RNA
ctcctcagtcgcggcttcct

SEQ ID NO: 10212 - RNA, 20 nt, synthetic construct
  source 1..20: mol_type = other RNA
gtaggggagctcctcagtcg

SEQ ID NO: 10213 - RNA, 20 nt, synthetic construct
  source 1..20: mol_type = other RNA
ctcccctaccctcccctttc

SEQ ID NO: 10214 - RNA, 20 nt, synthetic construct
  source 1..20: mol_type = other RNA
ggccggaaaggggagggtag

SEQ ID NO: 10215 - RNA, 20 nt, synthetic construct
  source 1..20: mol_type = other RNA
aggccggaaaggggagggta

SEQ ID NO: 10216 - RNA, 20 nt, synthetic construct
  source 1..20: mol_type = other RNA
gaggccggaaaggggagggt

SEQ ID NO: 10217 - RNA, 20 nt, synthetic construct
  source 1..20: mol_type = other RNA
tgcagaggccggaaagggga

SEQ ID NO: 10218 - RNA, 20 nt, synthetic construct
  source 1..20: mol_type = other RNA
ctgcagaggccggaaagggg

SEQ ID NO: 10219 - RNA, 20 nt, synthetic construct
  source 1..20: mol_type = other RNA
agtctgcagaggccggaaag

SEQ ID NO: 10220 - RNA, 20 nt, synthetic construct
  source 1..20: mol_type = other RNA
aagtctgcagaggccggaaa

SEQ ID NO: 10221 - RNA, 20 nt, synthetic construct
  source 1..20: mol_type = other RNA
aaagtctgcagaggccggaa

SEQ ID NO: 10222 - RNA, 20 nt, synthetic construct
  source 1..20: mol_type = other RNA
ggtgcaaagtctgcagaggc

SEQ ID NO: 10223 - RNA, 20 nt, synthetic construct
  source 1..20: mol_type = other RNA
gaatggtgcaaagtctgcag

SEQ ID NO: 10224 - RNA, 20 nt, synthetic construct
  source 1..20: mol_type = other RNA
cattccactccctccgctga

SEQ ID NO: 10225 - RNA, 20 nt, synthetic construct
  source 1..20: mol_type = other RNA
cgtcagcggagggagtggaa

SEQ ID NO: 10226 - RNA, 20 nt, synthetic construct
  source 1..20: mol_type = other RNA
tccctccgctgacggagaaa

SEQ ID NO: 10227 - RNA, 20 nt, synthetic construct
  source 1..20: mol_type = other RNA
ttctccgtcagcggagggag

SEQ ID NO: 10228 - RNA, 20 nt, synthetic construct
  source 1..20: mol_type = other RNA
tccttttctccgtcagcgga

SEQ ID NO: 10229 - RNA, 20 nt, synthetic construct
  source 1..20: mol_type = other RNA
ttccttttctccgtcagcgg

SEQ ID NO: 10230 - RNA, 20 nt, synthetic construct
  source 1..20: mol_type = other RNA
agtttccttttctccgtcag

SEQ ID NO: 10231 - RNA, 20 nt, synthetic construct
  source 1..20: mol_type = other RNA
aaaaggaaactttgtgtctg

SEQ ID NO: 10232 - RNA, 20 nt, synthetic construct
  source 1..20: mol_type = other RNA
ggaaactttgtgtctgcgga

SEQ ID NO: 10233 - RNA, 20 nt, synthetic construct
  source 1..20: mol_type = other RNA
gagagcctcccttgccaacg

SEQ ID NO: 10234 - RNA, 20 nt, synthetic construct
  source 1..20: mol_type = other RNA
agcctcccttgccaacgcgg

SEQ ID NO: 10235 - RNA, 20 nt, synthetic construct
  source 1..20: mol_type = other RNA
gcctcccttgccaacgcggt

SEQ ID NO: 10236 - RNA, 20 nt, synthetic construct
  source 1..20: mol_type = other RNA
tcccaccgcgttggcaaggg

SEQ ID NO: 10237 - RNA, 20 nt, synthetic construct
  source 1..20: mol_type = other RNA
tgccaacgcggtgggaacag

SEQ ID NO: 10238 - RNA, 20 nt, synthetic construct
  source 1..20: mol_type = other RNA
tgttcccaccgcgttggcaa

SEQ ID NO: 10239 - RNA, 20 nt, synthetic construct
  source 1..20: mol_type = other RNA
ctgttcccaccgcgttggca

SEQ ID NO: 10240 - RNA, 20 nt, synthetic construct
  source 1..20: mol_type = other RNA
cgcctctgttcccaccgcgt

SEQ ID NO: 10241 - RNA, 20 nt, synthetic construct
  source 1..20: mol_type = other RNA
ggaacagaggcgtacacgca

SEQ ID NO: 10242 - RNA, 20 nt, synthetic construct
  source 1..20: mol_type = other RNA
caccatccacagatacacgc

SEQ ID NO: 10243 - RNA, 20 nt, synthetic construct
  source 1..20: mol_type = other RNA
accatccacagatacacgca

SEQ ID NO: 10244 - RNA, 20 nt, synthetic construct
  source 1..20: mol_type = other RNA
accctgcgtgtatctgtgga

SEQ ID NO: 10245 - RNA, 20 nt, synthetic construct
  source 1..20: mol_type = other RNA
tgtgaccctgcgtgtatctg

SEQ ID NO: 10246 - RNA, 20 nt, synthetic construct
  source 1..20: mol_type = other RNA
ctgtgtttgtgtttctgagc

SEQ ID NO: 10247 - RNA, 20 nt, synthetic construct
  source 1..20: mol_type = other RNA
gcagtcgcacttacaagact

SEQ ID NO: 10248 - RNA, 20 nt, synthetic construct
  source 1..20: mol_type = other RNA
cacttacaagacttggtccc

SEQ ID NO: 10249 - RNA, 20 nt, synthetic construct
  source 1..20: mol_type = other RNA
acttacaagacttggtccca

SEQ ID NO: 10250 - RNA, 20 nt, synthetic construct
  source 1..20: mol_type = other RNA
acaagacttggtcccagggc

SEQ ID NO: 10251 - RNA, 20 nt, synthetic construct
  source 1..20: mol_type = other RNA
caagacttggtcccagggcc

SEQ ID NO: 10252 - RNA, 20 nt, synthetic construct
  source 1..20: mol_type = other RNA
tcccagggccgggcaccgag

SEQ ID NO: 10253 - RNA, 20 nt, synthetic construct
  source 1..20: mol_type = other RNA
gccactcggtgcccggccct

SEQ ID NO: 10254 - RNA, 20 nt, synthetic construct
  source 1..20: mol_type = other RNA
agccactcggtgcccggccc

SEQ ID NO: 10255 - RNA, 20 nt, synthetic construct
  source 1..20: mol_type = other RNA
aggcagagccactcggtgcc

SEQ ID NO: 10256 - RNA, 20 nt, synthetic construct
  source 1..20: mol_type = other RNA
ggatcgcaggcagagccact

SEQ ID NO: 10257 - RNA, 20 nt, synthetic construct
  source 1..20: mol_type = other RNA
ctgcctgcgatccagcactt

SEQ ID NO: 10258 - RNA, 20 nt, synthetic construct
  source 1..20: mol_type = other RNA
tgcctgcgatccagcacttt

SEQ ID NO: 10259 - RNA, 20 nt, synthetic construct
  source 1..20: mol_type = other RNA
ctgcgatccagcactttggg

SEQ ID NO: 10260 - RNA, 20 nt, synthetic construct
  source 1..20: mol_type = other RNA
ctcccaaagtgctggatcgc

SEQ ID NO: 10261 - RNA, 20 nt, synthetic construct
  source 1..20: mol_type = other RNA
tccagcactttgggaggccg

SEQ ID NO: 10262 - RNA, 20 nt, synthetic construct
  source 1..20: mol_type = other RNA
agcactttgggaggccgagg

SEQ ID NO: 10263 - RNA, 20 nt, synthetic construct
  source 1..20: mol_type = other RNA
gcactttgggaggccgaggc

SEQ ID NO: 10264 - RNA, 20 nt, synthetic construct
  source 1..20: mol_type = other RNA
gcctcggcctcccaaagtgc

SEQ ID NO: 10265 - RNA, 20 nt, synthetic construct
  source 1..20: mol_type = other RNA
ctttgggaggccgaggcggg

SEQ ID NO: 10266 - RNA, 20 nt, synthetic construct
  source 1..20: mol_type = other RNA
gccgaggcgggaggatcgct

SEQ ID NO: 10267 - RNA, 20 nt, synthetic construct
  source 1..20: mol_type = other RNA
ccgaggcgggaggatcgctt

SEQ ID NO: 10268 - RNA, 20 nt, synthetic construct
  source 1..20: mol_type = other RNA
cgaggcgggaggatcgcttg

SEQ ID NO: 10269 - RNA, 20 nt, synthetic construct
  source 1..20: mol_type = other RNA
cccaagcgatcctcccgcct

SEQ ID NO: 10270 - RNA, 20 nt, synthetic construct
  source 1..20: mol_type = other RNA
ccagaagtttgagagcagcc

SEQ ID NO: 10271 - RNA, 20 nt, synthetic construct
  source 1..20: mol_type = other RNA
cagaagtttgagagcagcct

SEQ ID NO: 10272 - RNA, 20 nt, synthetic construct
  source 1..20: mol_type = other RNA
ccaggctgctctcaaacttc

SEQ ID NO: 10273 - RNA, 20 nt, synthetic construct
  source 1..20: mol_type = other RNA
tgagagcagcctgggcaacg

SEQ ID NO: 10274 - RNA, 20 nt, synthetic construct
  source 1..20: mol_type = other RNA
agagtctcaccacgttgccc

SEQ ID NO: 10275 - RNA, 20 nt, synthetic construct
  source 1..20: mol_type = other RNA
aatttttttttgtagagaag

SEQ ID NO: 10276 - RNA, 20 nt, synthetic construct
  source 1..20: mol_type = other RNA
attgaaaagttagccaagtg

SEQ ID NO: 10277 - RNA, 20 nt, synthetic construct
  source 1..20: mol_type = other RNA
gaaaagttagccaagtgtgg

SEQ ID NO: 10278 - RNA, 20 nt, synthetic construct
  source 1..20: mol_type = other RNA
ctacaggcggccaccacact

SEQ ID NO: 10279 - RNA, 20 nt, synthetic construct
  source 1..20: mol_type = other RNA
cgcctgtagtcccagctgct

SEQ ID NO: 10280 - RNA, 20 nt, synthetic construct
  source 1..20: mol_type = other RNA
gcctgtagtcccagctgctt

SEQ ID NO: 10281 - RNA, 20 nt, synthetic construct
  source 1..20: mol_type = other RNA
caagcagctgggactacagg

SEQ ID NO: 10282 - RNA, 20 nt, synthetic construct
  source 1..20: mol_type = other RNA
tcccaagcagctgggactac

SEQ ID NO: 10283 - RNA, 20 nt, synthetic construct
  source 1..20: mol_type = other RNA
gctgcttgggaggatgagac

SEQ ID NO: 10284 - RNA, 20 nt, synthetic construct
  source 1..20: mol_type = other RNA
tctcatcctcccaagcagct

SEQ ID NO: 10285 - RNA, 20 nt, synthetic construct
  source 1..20: mol_type = other RNA
gtctcatcctcccaagcagc

SEQ ID NO: 10286 - RNA, 20 nt, synthetic construct
  source 1..20: mol_type = other RNA
gcttgggaggatgagacagg

SEQ ID NO: 10287 - RNA, 20 nt, synthetic construct
  source 1..20: mol_type = other RNA
caggaggatcgcttgagccc

SEQ ID NO: 10288 - RNA, 20 nt, synthetic construct
  source 1..20: mol_type = other RNA
gaggatcgcttgagccctgg

SEQ ID NO: 10289 - RNA, 20 nt, synthetic construct
  source 1..20: mol_type = other RNA
cgcttgagccctggaggtca

SEQ ID NO: 10290 - RNA, 20 nt, synthetic construct
  source 1..20: mol_type = other RNA
tgtgtgggctgcactgcccc

SEQ ID NO: 10291 - RNA, 20 nt, synthetic construct
  source 1..20: mol_type = other RNA
aggggcagtgcagcccacac

SEQ ID NO: 10292 - RNA, 20 nt, synthetic construct
  source 1..20: mol_type = other RNA
gggctgcactgcccctggtc

SEQ ID NO: 10293 - RNA, 20 nt, synthetic construct
  source 1..20: mol_type = other RNA
tgcactgcccctggtcaggc

SEQ ID NO: 10294 - RNA, 20 nt, synthetic construct
  source 1..20: mol_type = other RNA
gcccctggtcaggcaggcca

SEQ ID NO: 10295 - RNA, 20 nt, synthetic construct
  source 1..20: mol_type = other RNA
ctggtcaggcaggccatggt

SEQ ID NO: 10296 - RNA, 20 nt, synthetic construct
  source 1..20: mol_type = other RNA
accatggcctgcctgaccag

SEQ ID NO: 10297 - RNA, 20 nt, synthetic construct
  source 1..20: mol_type = other RNA
taccatggcctgcctgacca

SEQ ID NO: 10298 - RNA, 20 nt, synthetic construct
  source 1..20: mol_type = other RNA
ctaccatggcctgcctgacc

SEQ ID NO: 10299 - RNA, 20 nt, synthetic construct
  source 1..20: mol_type = other RNA
caggcaggccatggtaggag

SEQ ID NO: 10300 - RNA, 20 nt, synthetic construct
  source 1..20: mol_type = other RNA
aggccatggtaggagtggcc

SEQ ID NO: 10301 - RNA, 20 nt, synthetic construct
  source 1..20: mol_type = other RNA
atggtaggagtggcccggca

SEQ ID NO: 10302 - RNA, 20 nt, synthetic construct
  source 1..20: mol_type = other RNA
atgccgggccactcctacca

SEQ ID NO: 10303 - RNA, 20 nt, synthetic construct
  source 1..20: mol_type = other RNA
ggagtggcccggcatggccc

SEQ ID NO: 10304 - RNA, 20 nt, synthetic construct
  source 1..20: mol_type = other RNA
aagggctccggggccatgcc

SEQ ID NO: 10305 - RNA, 20 nt, synthetic construct
  source 1..20: mol_type = other RNA
gaagggctccggggccatgc

SEQ ID NO: 10306 - RNA, 20 nt, synthetic construct
  source 1..20: mol_type = other RNA
gaggggcaggaagggctccg

SEQ ID NO: 10307 - RNA, 20 nt, synthetic construct
  source 1..20: mol_type = other RNA
agaggggcaggaagggctcc

SEQ ID NO: 10308 - RNA, 20 nt, synthetic construct
  source 1..20: mol_type = other RNA
gagaggggcaggaagggctc

SEQ ID NO: 10309 - RNA, 20 nt, synthetic construct
  source 1..20: mol_type = other RNA
ttcctgcccctctctgatat

SEQ ID NO: 10310 - RNA, 20 nt, synthetic construct
  source 1..20: mol_type = other RNA
atatcagagaggggcaggaa

SEQ ID NO: 10311 - RNA, 20 nt, synthetic construct
  source 1..20: mol_type = other RNA
aatatcagagaggggcagga

SEQ ID NO: 10312 - RNA, 20 nt, synthetic construct
  source 1..20: mol_type = other RNA
gtccaatatcagagaggggc

SEQ ID NO: 10313 - RNA, 20 nt, synthetic construct
  source 1..20: mol_type = other RNA
aagggtccaatatcagagag

SEQ ID NO: 10314 - RNA, 20 nt, synthetic construct
  source 1..20: mol_type = other RNA
gaagggtccaatatcagaga

SEQ ID NO: 10315 - RNA, 20 nt, synthetic construct
  source 1..20: mol_type = other RNA
ggaagggtccaatatcagag

SEQ ID NO: 10316 - RNA, 20 nt, synthetic construct
  source 1..20: mol_type = other RNA
cttccctcatatgactccct

SEQ ID NO: 10317 - RNA, 20 nt, synthetic construct
  source 1..20: mol_type = other RNA
ttccctcatatgactcccta

SEQ ID NO: 10318 - RNA, 20 nt, synthetic construct
  source 1..20: mol_type = other RNA
tagggagtcatatgagggaa

SEQ ID NO: 10319 - RNA, 20 nt, synthetic construct
  source 1..20: mol_type = other RNA
ctagggagtcatatgaggga

SEQ ID NO: 10320 - RNA, 20 nt, synthetic construct
  source 1..20: mol_type = other RNA
agccctagggagtcatatga

SEQ ID NO: 10321 - RNA, 20 nt, synthetic construct
  source 1..20: mol_type = other RNA
cagccctagggagtcatatg

SEQ ID NO: 10322 - RNA, 20 nt, synthetic construct
  source 1..20: mol_type = other RNA
ggatgtcttgttcagcccta

SEQ ID NO: 10323 - RNA, 20 nt, synthetic construct
  source 1..20: mol_type = other RNA
aggatgtcttgttcagccct

SEQ ID NO: 10324 - RNA, 20 nt, synthetic construct
  source 1..20: mol_type = other RNA
atgggcttcgcaggagaaag

SEQ ID NO: 10325 - RNA, 20 nt, synthetic construct
  source 1..20: mol_type = other RNA
ctgcgaagcccataacgcca

SEQ ID NO: 10326 - RNA, 20 nt, synthetic construct
  source 1..20: mol_type = other RNA
tgcgaagcccataacgccaa

SEQ ID NO: 10327 - RNA, 20 nt, synthetic construct
  source 1..20: mol_type = other RNA
gcgaagcccataacgccaag

SEQ ID NO: 10328 - RNA, 20 nt, synthetic construct
  source 1..20: mol_type = other RNA
cgaagcccataacgccaagg

SEQ ID NO: 10329 - RNA, 20 nt, synthetic construct
  source 1..20: mol_type = other RNA
cttggcgttatgggcttcgc

SEQ ID NO: 10330 - RNA, 20 nt, synthetic construct
  source 1..20: mol_type = other RNA
ggtgacccccttggcgttat

SEQ ID NO: 10331 - RNA, 20 nt, synthetic construct
  source 1..20: mol_type = other RNA
tggtgacccccttggcgtta

SEQ ID NO: 10332 - RNA, 20 nt, synthetic construct
  source 1..20: mol_type = other RNA
gcgggatgtggtgaccccct

SEQ ID NO: 10333 - RNA, 20 nt, synthetic construct
  source 1..20: mol_type = other RNA
tcccgcacagccaccatcac

SEQ ID NO: 10334 - RNA, 20 nt, synthetic construct
  source 1..20: mol_type = other RNA
acctgtgatggtggctgtgc

SEQ ID NO: 10335 - RNA, 20 nt, synthetic construct
  source 1..20: mol_type = other RNA
cacctgtgatggtggctgtg

SEQ ID NO: 10336 - RNA, 20 nt, synthetic construct
  source 1..20: mol_type = other RNA
accatcacaggtgacagagt

SEQ ID NO: 10337 - RNA, 20 nt, synthetic construct
  source 1..20: mol_type = other RNA
ccatcacaggtgacagagtt

SEQ ID NO: 10338 - RNA, 20 nt, synthetic construct
  source 1..20: mol_type = other RNA
aactctgtcacctgtgatgg

SEQ ID NO: 10339 - RNA, 20 nt, synthetic construct
  source 1..20: mol_type = other RNA
tcacaggtgacagagttggg

SEQ ID NO: 10340 - RNA, 20 nt, synthetic construct
  source 1..20: mol_type = other RNA
cccaactctgtcacctgtga

SEQ ID NO: 10341 - RNA, 20 nt, synthetic construct
  source 1..20: mol_type = other RNA
caggtgacagagttgggagg

SEQ ID NO: 10342 - RNA, 20 nt, synthetic construct
  source 1..20: mol_type = other RNA
aggtgacagagttgggaggt

SEQ ID NO: 10343 - RNA, 20 nt, synthetic construct
  source 1..20: mol_type = other RNA
ggtgacagagttgggaggtg

SEQ ID NO: 10344 - RNA, 20 nt, synthetic construct
  source 1..20: mol_type = other RNA
agagttgggaggtggggagc

SEQ ID NO: 10345 - RNA, 20 nt, synthetic construct
  source 1..20: mol_type = other RNA
gagttgggaggtggggagct

SEQ ID NO: 10346 - RNA, 20 nt, synthetic construct
  source 1..20: mol_type = other RNA
ggtggggagctgggcgtcag

SEQ ID NO: 10347 - RNA, 20 nt, synthetic construct
  source 1..20: mol_type = other RNA
gtggggagctgggcgtcaga

SEQ ID NO: 10348 - RNA, 20 nt, synthetic construct
  source 1..20: mol_type = other RNA
gggagctgggcgtcagaggg

SEQ ID NO: 10349 - RNA, 20 nt, synthetic construct
  source 1..20: mol_type = other RNA
ggagctgggcgtcagagggt

SEQ ID NO: 10350 - RNA, 20 nt, synthetic construct
  source 1..20: mol_type = other RNA
gagctgggcgtcagagggtg

SEQ ID NO: 10351 - RNA, 20 nt, synthetic construct
  source 1..20: mol_type = other RNA
gggcgtcagagggtggggtt

SEQ ID NO: 10352 - RNA, 20 nt, synthetic construct
  source 1..20: mol_type = other RNA
ggcgtcagagggtggggttt

SEQ ID NO: 10353 - RNA, 20 nt, synthetic construct
  source 1..20: mol_type = other RNA
cagagggtggggtttgggtc

SEQ ID NO: 10354 - RNA, 20 nt, synthetic construct
  source 1..20: mol_type = other RNA
agagggtggggtttgggtcc

SEQ ID NO: 10355 - RNA, 20 nt, synthetic construct
  source 1..20: mol_type = other RNA
gagggtggggtttgggtccg

SEQ ID NO: 10356 - RNA, 20 nt, synthetic construct
  source 1..20: mol_type = other RNA
gtttgggtccggggtcagag

SEQ ID NO: 10357 - RNA, 20 nt, synthetic construct
  source 1..20: mol_type = other RNA
tttgggtccggggtcagagt

SEQ ID NO: 10358 - RNA, 20 nt, synthetic construct
  source 1..20: mol_type = other RNA
ttgggtccggggtcagagtg

SEQ ID NO: 10359 - RNA, 20 nt, synthetic construct
  source 1..20: mol_type = other RNA
tgggtccggggtcagagtgg

SEQ ID NO: 10360 - RNA, 20 nt, synthetic construct
  source 1..20: mol_type = other RNA
ctctgcccccactctgaccc

SEQ ID NO: 10361 - RNA, 20 nt, synthetic construct
  source 1..20: mol_type = other RNA
tcagagtgggggcagagagc

SEQ ID NO: 10362 - RNA, 20 nt, synthetic construct
  source 1..20: mol_type = other RNA
cagagtgggggcagagagca

SEQ ID NO: 10363 - RNA, 20 nt, synthetic construct
  source 1..20: mol_type = other RNA
gtgggggcagagagcagggt

SEQ ID NO: 10364 - RNA, 20 nt, synthetic construct
  source 1..20: mol_type = other RNA
tgggggcagagagcagggta

SEQ ID NO: 10365 - RNA, 20 nt, synthetic construct
  source 1..20: mol_type = other RNA
gggtagggagctttgagcaa

SEQ ID NO: 10366 - RNA, 20 nt, synthetic construct
  source 1..20: mol_type = other RNA
gctttgagcaaaggctcccc

SEQ ID NO: 10367 - RNA, 20 nt, synthetic construct
  source 1..20: mol_type = other RNA
ctttgagcaaaggctcccca

SEQ ID NO: 10368 - RNA, 20 nt, synthetic construct
  source 1..20: mol_type = other RNA
aacgggagagattgaccctg

SEQ ID NO: 10369 - RNA, 20 nt, synthetic construct
  source 1..20: mol_type = other RNA
aaacgggagagattgaccct

SEQ ID NO: 10370 - RNA, 20 nt, synthetic construct
  source 1..20: mol_type = other RNA
caaacgggagagattgaccc

SEQ ID NO: 10371 - RNA, 20 nt, synthetic construct
  source 1..20: mol_type = other RNA
ggggagcactgtggacaaac

SEQ ID NO: 10372 - RNA, 20 nt, synthetic construct
  source 1..20: mol_type = other RNA
gggggagcactgtggacaaa

SEQ ID NO: 10373 - RNA, 20 nt, synthetic construct
  source 1..20: mol_type = other RNA
gggctgctgggggagcactg

SEQ ID NO: 10374 - RNA, 20 nt, synthetic construct
  source 1..20: mol_type = other RNA
ggaggttacggggctgctgg

SEQ ID NO: 10375 - RNA, 20 nt, synthetic construct
  source 1..20: mol_type = other RNA
gcagccccgtaacctccacc

SEQ ID NO: 10376 - RNA, 20 nt, synthetic construct
  source 1..20: mol_type = other RNA
gtggaggttacggggctgct

SEQ ID NO: 10377 - RNA, 20 nt, synthetic construct
  source 1..20: mol_type = other RNA
ggtggaggttacggggctgc

SEQ ID NO: 10378 - RNA, 20 nt, synthetic construct
  source 1..20: mol_type = other RNA
gagaccaggtggaggttacg

SEQ ID NO: 10379 - RNA, 20 nt, synthetic construct
  source 1..20: mol_type = other RNA
ggagaccaggtggaggttac

SEQ ID NO: 10380 - RNA, 20 nt, synthetic construct
  source 1..20: mol_type = other RNA
gggagaccaggtggaggtta

SEQ ID NO: 10381 - RNA, 20 nt, synthetic construct
  source 1..20: mol_type = other RNA
gttggcgggagaccaggtgg

SEQ ID NO: 10382 - RNA, 20 nt, synthetic construct
  source 1..20: mol_type = other RNA
cctggtctcccgccaaccca

SEQ ID NO: 10383 - RNA, 20 nt, synthetic construct
  source 1..20: mol_type = other RNA
tgggttggcgggagaccagg

SEQ ID NO: 10384 - RNA, 20 nt, synthetic construct
  source 1..20: mol_type = other RNA
ccgtgggttggcgggagacc

SEQ ID NO: 10385 - RNA, 20 nt, synthetic construct
  source 1..20: mol_type = other RNA
ctcccgccaacccacggagc

SEQ ID NO: 10386 - RNA, 20 nt, synthetic construct
  source 1..20: mol_type = other RNA
ccgccaacccacggagctgg

SEQ ID NO: 10387 - RNA, 20 nt, synthetic construct
  source 1..20: mol_type = other RNA
ccaacccacggagctggagg

SEQ ID NO: 10388 - RNA, 20 nt, synthetic construct
  source 1..20: mol_type = other RNA
ctccagctccgtgggttggc

SEQ ID NO: 10389 - RNA, 20 nt, synthetic construct
  source 1..20: mol_type = other RNA
cctccagctccgtgggttgg

SEQ ID NO: 10390 - RNA, 20 nt, synthetic construct
  source 1..20: mol_type = other RNA
ccacggagctggaggtggct

SEQ ID NO: 10391 - RNA, 20 nt, synthetic construct
  source 1..20: mol_type = other RNA
caagccacctccagctccgt

SEQ ID NO: 10392 - RNA, 20 nt, synthetic construct
  source 1..20: mol_type = other RNA
ccaagccacctccagctccg

SEQ ID NO: 10393 - RNA, 20 nt, synthetic construct
  source 1..20: mol_type = other RNA
ctggaggtggcttggactcc

SEQ ID NO: 10394 - RNA, 20 nt, synthetic construct
  source 1..20: mol_type = other RNA
gcttggactccaggcctgag

SEQ ID NO: 10395 - RNA, 20 nt, synthetic construct
  source 1..20: mol_type = other RNA
gggtagatgccgctcaggcc

SEQ ID NO: 10396 - RNA, 20 nt, synthetic construct
  source 1..20: mol_type = other RNA
tcagggggtagatgccgctc

SEQ ID NO: 10397 - RNA, 20 nt, synthetic construct
  source 1..20: mol_type = other RNA
cctgacccactgcaccctgc

SEQ ID NO: 10398 - RNA, 20 nt, synthetic construct
  source 1..20: mol_type = other RNA
gcagggtgcagtgggtcagg

SEQ ID NO: 10399 - RNA, 20 nt, synthetic construct
  source 1..20: mol_type = other RNA
tgcagggtgcagtgggtcag

SEQ ID NO: 10400 - RNA, 20 nt, synthetic construct
  source 1..20: mol_type = other RNA
ctgcagggtgcagtgggtca

SEQ ID NO: 10401 - RNA, 20 nt, synthetic construct
  source 1..20: mol_type = other RNA
cctgcagggtgcagtgggtc

SEQ ID NO: 10402 - RNA, 20 nt, synthetic construct
  source 1..20: mol_type = other RNA
tctcacctgcagggtgcagt

SEQ ID NO: 10403 - RNA, 20 nt, synthetic construct
  source 1..20: mol_type = other RNA
gtctcacctgcagggtgcag

SEQ ID NO: 10404 - RNA, 20 nt, synthetic construct
  source 1..20: mol_type = other RNA
gcaggtgagactcccaaact

SEQ ID NO: 10405 - RNA, 20 nt, synthetic construct
  source 1..20: mol_type = other RNA
gtttgggagtctcacctgca

SEQ ID NO: 10406 - RNA, 20 nt, synthetic construct
  source 1..20: mol_type = other RNA
agtttgggagtctcacctgc

SEQ ID NO: 10407 - RNA, 20 nt, synthetic construct
  source 1..20: mol_type = other RNA
acttggttcatttcagtctc

SEQ ID NO: 10408 - RNA, 20 nt, synthetic construct
  source 1..20: mol_type = other RNA
agactgaaatgaaccaagtt

SEQ ID NO: 10409 - RNA, 20 nt, synthetic construct
  source 1..20: mol_type = other RNA
ttgtggatgtgggtggaagg

SEQ ID NO: 10410 - RNA, 20 nt, synthetic construct
  source 1..20: mol_type = other RNA
gggttgtggatgtgggtgga

SEQ ID NO: 10411 - RNA, 20 nt, synthetic construct
  source 1..20: mol_type = other RNA
atgggggttgtggatgtggg

SEQ ID NO: 10412 - RNA, 20 nt, synthetic construct
  source 1..20: mol_type = other RNA
aggatgggggttgtggatgt

SEQ ID NO: 10413 - RNA, 20 nt, synthetic construct
  source 1..20: mol_type = other RNA
gaggatgggggttgtggatg

SEQ ID NO: 10414 - RNA, 20 nt, synthetic construct
  source 1..20: mol_type = other RNA
cacaacccccatcctctccc

SEQ ID NO: 10415 - RNA, 20 nt, synthetic construct
  source 1..20: mol_type = other RNA
acaacccccatcctctccct

SEQ ID NO: 10416 - RNA, 20 nt, synthetic construct
  source 1..20: mol_type = other RNA
cagggagaggatgggggttg

SEQ ID NO: 10417 - RNA, 20 nt, synthetic construct
  source 1..20: mol_type = other RNA
ggttcccagggagaggatgg

SEQ ID NO: 10418 - RNA, 20 nt, synthetic construct
  source 1..20: mol_type = other RNA
gggttcccagggagaggatg

SEQ ID NO: 10419 - RNA, 20 nt, synthetic construct
  source 1..20: mol_type = other RNA
tgggttcccagggagaggat

SEQ ID NO: 10420 - RNA, 20 nt, synthetic construct
  source 1..20: mol_type = other RNA
gtgggttcccagggagagga

SEQ ID NO: 10421 - RNA, 20 nt, synthetic construct
  source 1..20: mol_type = other RNA
agtggtgggttcccagggag

SEQ ID NO: 10422 - RNA, 20 nt, synthetic construct
  source 1..20: mol_type = other RNA
cctgggaacccaccacttct

SEQ ID NO: 10423 - RNA, 20 nt, synthetic construct
  source 1..20: mol_type = other RNA
cgagaagtggtgggttccca

SEQ ID NO: 10424 - RNA, 20 nt, synthetic construct
  source 1..20: mol_type = other RNA
ccgagaagtggtgggttccc

SEQ ID NO: 10425 - RNA, 20 nt, synthetic construct
  source 1..20: mol_type = other RNA
aacagtggccgagaagtggt

SEQ ID NO: 10426 - RNA, 20 nt, synthetic construct
  source 1..20: mol_type = other RNA
caacagtggccgagaagtgg

SEQ ID NO: 10427 - RNA, 20 nt, synthetic construct
  source 1..20: mol_type = other RNA
tctcaacagtggccgagaag

SEQ ID NO: 10428 - RNA, 20 nt, synthetic construct
  source 1..20: mol_type = other RNA
tgttgagaagcagtagagcc

SEQ ID NO: 10429 - RNA, 20 nt, synthetic construct
  source 1..20: mol_type = other RNA
gttgagaagcagtagagcct

SEQ ID NO: 10430 - RNA, 20 nt, synthetic construct
  source 1..20: mol_type = other RNA
ttgagaagcagtagagcctg

SEQ ID NO: 10431 - RNA, 20 nt, synthetic construct
  source 1..20: mol_type = other RNA
tgagaagcagtagagcctgg

SEQ ID NO: 10432 - RNA, 20 nt, synthetic construct
  source 1..20: mol_type = other RNA
gagaagcagtagagcctggg

SEQ ID NO: 10433 - RNA, 20 nt, synthetic construct
  source 1..20: mol_type = other RNA
gtgactacacaacttttcaa

SEQ ID NO: 10434 - RNA, 20 nt, synthetic construct
  source 1..20: mol_type = other RNA
tgtgactacacaacttttca

SEQ ID NO: 10435 - RNA, 20 nt, synthetic construct
  source 1..20: mol_type = other RNA
tcacaccagaccaccaccac

SEQ ID NO: 10436 - RNA, 20 nt, synthetic construct
  source 1..20: mol_type = other RNA
cacaccagaccaccaccact

SEQ ID NO: 10437 - RNA, 20 nt, synthetic construct
  source 1..20: mol_type = other RNA
agctcccagtggtggtggtc

SEQ ID NO: 10438 - RNA, 20 nt, synthetic construct
  source 1..20: mol_type = other RNA
cacacagctcccagtggtgg

SEQ ID NO: 10439 - RNA, 20 nt, synthetic construct
  source 1..20: mol_type = other RNA
ggtcacacagctcccagtgg

SEQ ID NO: 10440 - RNA, 20 nt, synthetic construct
  source 1..20: mol_type = other RNA
gatggtcacacagctcccag

SEQ ID NO: 10441 - RNA, 20 nt, synthetic construct
  source 1..20: mol_type = other RNA
gaccatctcgtgtgattgct

SEQ ID NO: 10442 - RNA, 20 nt, synthetic construct
  source 1..20: mol_type = other RNA
agccaagcaatcacacgaga

SEQ ID NO: 10443 - RNA, 20 nt, synthetic construct
  source 1..20: mol_type = other RNA
agaggcaagggtgtgaggac

SEQ ID NO: 10444 - RNA, 20 nt, synthetic construct
  source 1..20: mol_type = other RNA
gagaggcaagggtgtgagga

SEQ ID NO: 10445 - RNA, 20 nt, synthetic construct
  source 1..20: mol_type = other RNA
tcacacccttgcctctcctc

SEQ ID NO: 10446 - RNA, 20 nt, synthetic construct
  source 1..20: mol_type = other RNA
tgaggagaggcaagggtgtg

SEQ ID NO: 10447 - RNA, 20 nt, synthetic construct
  source 1..20: mol_type = other RNA
cacagcctgaggagaggcaa

SEQ ID NO: 10448 - RNA, 20 nt, synthetic construct
  source 1..20: mol_type = other RNA
gcacagcctgaggagaggca

SEQ ID NO: 10449 - RNA, 20 nt, synthetic construct
  source 1..20: mol_type = other RNA
tgacagcacagcctgaggag

SEQ ID NO: 10450 - RNA, 20 nt, synthetic construct
  source 1..20: mol_type = other RNA
caggctgtgctgtcagacga

SEQ ID NO: 10451 - RNA, 20 nt, synthetic construct
  source 1..20: mol_type = other RNA
aggctgtgctgtcagacgat

SEQ ID NO: 10452 - RNA, 20 nt, synthetic construct
  source 1..20: mol_type = other RNA
tcgtctgacagcacagcctg

SEQ ID NO: 10453 - RNA, 20 nt, synthetic construct
  source 1..20: mol_type = other RNA
tgtgctgtcagacgatggga

SEQ ID NO: 10454 - RNA, 20 nt, synthetic construct
  source 1..20: mol_type = other RNA
gtgctgtcagacgatgggat

SEQ ID NO: 10455 - RNA, 20 nt, synthetic construct
  source 1..20: mol_type = other RNA
agacgatgggatgggcatcc

SEQ ID NO: 10456 - RNA, 20 nt, synthetic construct
  source 1..20: mol_type = other RNA
cgatgggatgggcatccagg

SEQ ID NO: 10457 - RNA, 20 nt, synthetic construct
  source 1..20: mol_type = other RNA
gatgggatgggcatccaggc

SEQ ID NO: 10458 - RNA, 20 nt, synthetic construct
  source 1..20: mol_type = other RNA
gggggtctggttctcccgcc

SEQ ID NO: 10459 - RNA, 20 nt, synthetic construct
  source 1..20: mol_type = other RNA
gggagaaccagaccccccag

SEQ ID NO: 10460 - RNA, 20 nt, synthetic construct
  source 1..20: mol_type = other RNA
aggggctcctctggggggtc

SEQ ID NO: 10461 - RNA, 20 nt, synthetic construct
  source 1..20: mol_type = other RNA
aggtgaggggctcctctggg

SEQ ID NO: 10462 - RNA, 20 nt, synthetic construct
  source 1..20: mol_type = other RNA
gaggtgaggggctcctctgg

SEQ ID NO: 10463 - RNA, 20 nt, synthetic construct
  source 1..20: mol_type = other RNA
cgaggtgaggggctcctctg

SEQ ID NO: 10464 - RNA, 20 nt, synthetic construct
  source 1..20: mol_type = other RNA
gcgaggtgaggggctcctct

SEQ ID NO: 10465 - RNA, 20 nt, synthetic construct
  source 1..20: mol_type = other RNA
tgcgaggtgaggggctcctc

SEQ ID NO: 10466 - RNA, 20 nt, synthetic construct
  source 1..20: mol_type = other RNA
acggatgcttgcgaggtgag

SEQ ID NO: 10467 - RNA, 20 nt, synthetic construct
  source 1..20: mol_type = other RNA
cacggatgcttgcgaggtga

SEQ ID NO: 10468 - RNA, 20 nt, synthetic construct
  source 1..20: mol_type = other RNA
gcacggatgcttgcgaggtg

SEQ ID NO: 10469 - RNA, 20 nt, synthetic construct
  source 1..20: mol_type = other RNA
ggggggcacggatgcttgcg

SEQ ID NO: 10470 - RNA, 20 nt, synthetic construct
  source 1..20: mol_type = other RNA
ccgtgcccccccatcagctt

SEQ ID NO: 10471 - RNA, 20 nt, synthetic construct
  source 1..20: mol_type = other RNA
ccgaagctgatgggggggca

SEQ ID NO: 10472 - RNA, 20 nt, synthetic construct
  source 1..20: mol_type = other RNA
cctagccgaagctgatgggg

SEQ ID NO: 10473 - RNA, 20 nt, synthetic construct
  source 1..20: mol_type = other RNA
gcctagccgaagctgatggg

SEQ ID NO: 10474 - RNA, 20 nt, synthetic construct
  source 1..20: mol_type = other RNA
tgcctagccgaagctgatgg

SEQ ID NO: 10475 - RNA, 20 nt, synthetic construct
  source 1..20: mol_type = other RNA
ctgcctagccgaagctgatg

SEQ ID NO: 10476 - RNA, 20 nt, synthetic construct
  source 1..20: mol_type = other RNA
gctgcctagccgaagctgat

SEQ ID NO: 10477 - RNA, 20 nt, synthetic construct
  source 1..20: mol_type = other RNA
ggctgcctagccgaagctga

SEQ ID NO: 10478 - RNA, 20 nt, synthetic construct
  source 1..20: mol_type = other RNA
gataaggggtgtgaggatgg

SEQ ID NO: 10479 - RNA, 20 nt, synthetic construct
  source 1..20: mol_type = other RNA
tgtgataaggggtgtgagga

SEQ ID NO: 10480 - RNA, 20 nt, synthetic construct
  source 1..20: mol_type = other RNA
caccccttatcacatccgcg

SEQ ID NO: 10481 - RNA, 20 nt, synthetic construct
  source 1..20: mol_type = other RNA
tgccacgcggatgtgataag

SEQ ID NO: 10482 - RNA, 20 nt, synthetic construct
  source 1..20: mol_type = other RNA
atgccacgcggatgtgataa

SEQ ID NO: 10483 - RNA, 20 nt, synthetic construct
  source 1..20: mol_type = other RNA
catgccacgcggatgtgata

SEQ ID NO: 10484 - RNA, 20 nt, synthetic construct
  source 1..20: mol_type = other RNA
cgtggcatgcaccagcagcc

SEQ ID NO: 10485 - RNA, 20 nt, synthetic construct
  source 1..20: mol_type = other RNA
gtggcatgcaccagcagcca

SEQ ID NO: 10486 - RNA, 20 nt, synthetic construct
  source 1..20: mol_type = other RNA
ggctgctggtgcatgccacg

SEQ ID NO: 10487 - RNA, 20 nt, synthetic construct
  source 1..20: mol_type = other RNA
gcagccagggcccctcatcc

SEQ ID NO: 10488 - RNA, 20 nt, synthetic construct
  source 1..20: mol_type = other RNA
ggatgaggggccctggctgc

SEQ ID NO: 10489 - RNA, 20 nt, synthetic construct
  source 1..20: mol_type = other RNA
gggtccaggatgaggggccc

SEQ ID NO: 10490 - RNA, 20 nt, synthetic construct
  source 1..20: mol_type = other RNA
gccagtgggtccaggatgag

SEQ ID NO: 10491 - RNA, 20 nt, synthetic construct
  source 1..20: mol_type = other RNA
agccagtgggtccaggatga

SEQ ID NO: 10492 - RNA, 20 nt, synthetic construct
  source 1..20: mol_type = other RNA
aagccagtgggtccaggatg

SEQ ID NO: 10493 - RNA, 20 nt, synthetic construct
  source 1..20: mol_type = other RNA
ctggacccactggcttcctg

SEQ ID NO: 10494 - RNA, 20 nt, synthetic construct
  source 1..20: mol_type = other RNA
cacaggaagccagtgggtcc

SEQ ID NO: 10495 - RNA, 20 nt, synthetic construct
  source 1..20: mol_type = other RNA
ctggcttcctgtggagacgc

SEQ ID NO: 10496 - RNA, 20 nt, synthetic construct
  source 1..20: mol_type = other RNA
cgtctccacaggaagccagt

SEQ ID NO: 10497 - RNA, 20 nt, synthetic construct
  source 1..20: mol_type = other RNA
gcgtctccacaggaagccag

SEQ ID NO: 10498 - RNA, 20 nt, synthetic construct
  source 1..20: mol_type = other RNA
gcttcctgtggagacgccgg

SEQ ID NO: 10499 - RNA, 20 nt, synthetic construct
  source 1..20: mol_type = other RNA
cttcctgtggagacgccgga

SEQ ID NO: 10500 - RNA, 20 nt, synthetic construct
  source 1..20: mol_type = other RNA
cctgtggagacgccggaggg

SEQ ID NO: 10501 - RNA, 20 nt, synthetic construct
  source 1..20: mol_type = other RNA
cctccctccggcgtctccac

SEQ ID NO: 10502 - RNA, 20 nt, synthetic construct
  source 1..20: mol_type = other RNA
gacgccggagggaggtaaga

SEQ ID NO: 10503 - RNA, 20 nt, synthetic construct
  source 1..20: mol_type = other RNA
acgccggagggaggtaagaa

SEQ ID NO: 10504 - RNA, 20 nt, synthetic construct
  source 1..20: mol_type = other RNA
cggagggaggtaagaagggt

SEQ ID NO: 10505 - RNA, 20 nt, synthetic construct
  source 1..20: mol_type = other RNA
ggagggaggtaagaagggtt

SEQ ID NO: 10506 - RNA, 20 nt, synthetic construct
  source 1..20: mol_type = other RNA
gagggaggtaagaagggttg

SEQ ID NO: 10507 - RNA, 20 nt, synthetic construct
  source 1..20: mol_type = other RNA
caacccttcttacctccctc

SEQ ID NO: 10508 - RNA, 20 nt, synthetic construct
  source 1..20: mol_type = other RNA
ggaggtaagaagggttgggg

SEQ ID NO: 10509 - RNA, 20 nt, synthetic construct
  source 1..20: mol_type = other RNA
gaggtaagaagggttgggga

SEQ ID NO: 10510 - RNA, 20 nt, synthetic construct
  source 1..20: mol_type = other RNA
acacgtcaccactgccccac

SEQ ID NO: 10511 - RNA, 20 nt, synthetic construct
  source 1..20: mol_type = other RNA
agcaaggtccggtggggcag

SEQ ID NO: 10512 - RNA, 20 nt, synthetic construct
  source 1..20: mol_type = other RNA
gatataagcaaggtccggtg

SEQ ID NO: 10513 - RNA, 20 nt, synthetic construct
  source 1..20: mol_type = other RNA
tgatataagcaaggtccggt

SEQ ID NO: 10514 - RNA, 20 nt, synthetic construct
  source 1..20: mol_type = other RNA
ctgatataagcaaggtccgg

SEQ ID NO: 10515 - RNA, 20 nt, synthetic construct
  source 1..20: mol_type = other RNA
gcactgatataagcaaggtc

SEQ ID NO: 10516 - RNA, 20 nt, synthetic construct
  source 1..20: mol_type = other RNA
gggtggcactgatataagca

SEQ ID NO: 10517 - RNA, 20 nt, synthetic construct
  source 1..20: mol_type = other RNA
gtgaaaggggacaatggggg

SEQ ID NO: 10518 - RNA, 20 nt, synthetic construct
  source 1..20: mol_type = other RNA
ggagtgaaaggggacaatgg

SEQ ID NO: 10519 - RNA, 20 nt, synthetic construct
  source 1..20: mol_type = other RNA
aggagtgaaaggggacaatg

SEQ ID NO: 10520 - RNA, 20 nt, synthetic construct
  source 1..20: mol_type = other RNA
aaggagtgaaaggggacaat

SEQ ID NO: 10521 - RNA, 20 nt, synthetic construct
  source 1..20: mol_type = other RNA
aaaggagtgaaaggggacaa

SEQ ID NO: 10522 - RNA, 20 nt, synthetic construct
  source 1..20: mol_type = other RNA
tttcactcctttacccctca

SEQ ID NO: 10523 - RNA, 20 nt, synthetic construct
  source 1..20: mol_type = other RNA
gaggggtaaaggagtgaaag

SEQ ID NO: 10524 - RNA, 20 nt, synthetic construct
  source 1..20: mol_type = other RNA
tgaggggtaaaggagtgaaa

SEQ ID NO: 10525 - RNA, 20 nt, synthetic construct
  source 1..20: mol_type = other RNA
atgaggggtaaaggagtgaa

SEQ ID NO: 10526 - RNA, 20 nt, synthetic construct
  source 1..20: mol_type = other RNA
attgaggccatgaggggtaa

SEQ ID NO: 10527 - RNA, 20 nt, synthetic construct
  source 1..20: mol_type = other RNA
aaggagattgaggccatgag

SEQ ID NO: 10528 - RNA, 20 nt, synthetic construct
  source 1..20: mol_type = other RNA
gaaggagattgaggccatga

SEQ ID NO: 10529 - RNA, 20 nt, synthetic construct
  source 1..20: mol_type = other RNA
ggaaggagattgaggccatg

SEQ ID NO: 10530 - RNA, 20 nt, synthetic construct
  source 1..20: mol_type = other RNA
cacacgtgggcaactcgtgc

SEQ ID NO: 10531 - RNA, 20 nt, synthetic construct
  source 1..20: mol_type = other RNA
gttgcccacgtgtgtgccct

SEQ ID NO: 10532 - RNA, 20 nt, synthetic construct
  source 1..20: mol_type = other RNA
ggtgccaagggcacacacgt

SEQ ID NO: 10533 - RNA, 20 nt, synthetic construct
  source 1..20: mol_type = other RNA
gggtgccaagggcacacacg

SEQ ID NO: 10534 - RNA, 20 nt, synthetic construct
  source 1..20: mol_type = other RNA
aagtgggtgcagggtgccaa

SEQ ID NO: 10535 - RNA, 20 nt, synthetic construct
  source 1..20: mol_type = other RNA
gaagtgggtgcagggtgcca

SEQ ID NO: 10536 - RNA, 20 nt, synthetic construct
  source 1..20: mol_type = other RNA
tgcacccacttcctgggaac

SEQ ID NO: 10537 - RNA, 20 nt, synthetic construct
  source 1..20: mol_type = other RNA
gcacccacttcctgggaaca

SEQ ID NO: 10538 - RNA, 20 nt, synthetic construct
  source 1..20: mol_type = other RNA
gttcccaggaagtgggtgca

SEQ ID NO: 10539 - RNA, 20 nt, synthetic construct
  source 1..20: mol_type = other RNA
tgttcccaggaagtgggtgc

SEQ ID NO: 10540 - RNA, 20 nt, synthetic construct
  source 1..20: mol_type = other RNA
ccacttcctgggaacagggg

SEQ ID NO: 10541 - RNA, 20 nt, synthetic construct
  source 1..20: mol_type = other RNA
cacttcctgggaacagggga

SEQ ID NO: 10542 - RNA, 20 nt, synthetic construct
  source 1..20: mol_type = other RNA
acttcctgggaacaggggag

SEQ ID NO: 10543 - RNA, 20 nt, synthetic construct
  source 1..20: mol_type = other RNA
cttcctgggaacaggggagg

SEQ ID NO: 10544 - RNA, 20 nt, synthetic construct
  source 1..20: mol_type = other RNA
ctcccctgttcccaggaagt

SEQ ID NO: 10545 - RNA, 20 nt, synthetic construct
  source 1..20: mol_type = other RNA
cctcccctgttcccaggaag

SEQ ID NO: 10546 - RNA, 20 nt, synthetic construct
  source 1..20: mol_type = other RNA
tgggaacaggggagggggtc

SEQ ID NO: 10547 - RNA, 20 nt, synthetic construct
  source 1..20: mol_type = other RNA
tgaccccctcccctgttccc

SEQ ID NO: 10548 - RNA, 20 nt, synthetic construct
  source 1..20: mol_type = other RNA
caggggagggggtcaggaag

SEQ ID NO: 10549 - RNA, 20 nt, synthetic construct
  source 1..20: mol_type = other RNA
gggagggggtcaggaagagg

SEQ ID NO: 10550 - RNA, 20 nt, synthetic construct
  source 1..20: mol_type = other RNA
ggagggggtcaggaagaggt

SEQ ID NO: 10551 - RNA, 20 nt, synthetic construct
  source 1..20: mol_type = other RNA
gagggggtcaggaagaggtg

SEQ ID NO: 10552 - RNA, 20 nt, synthetic construct
  source 1..20: mol_type = other RNA
agggggtcaggaagaggtgg

SEQ ID NO: 10553 - RNA, 20 nt, synthetic construct
  source 1..20: mol_type = other RNA
ggacagggaagaggggaagc

SEQ ID NO: 10554 - RNA, 20 nt, synthetic construct
  source 1..20: mol_type = other RNA
cactggaggacagggaagag

SEQ ID NO: 10555 - RNA, 20 nt, synthetic construct
  source 1..20: mol_type = other RNA
gcactggaggacagggaaga

SEQ ID NO: 10556 - RNA, 20 nt, synthetic construct
  source 1..20: mol_type = other RNA
ggcactggaggacagggaag

SEQ ID NO: 10557 - RNA, 20 nt, synthetic construct
  source 1..20: mol_type = other RNA
ccctgtcctccagtgcccct

SEQ ID NO: 10558 - RNA, 20 nt, synthetic construct
  source 1..20: mol_type = other RNA
cccaggggcactggaggaca

SEQ ID NO: 10559 - RNA, 20 nt, synthetic construct
  source 1..20: mol_type = other RNA
gcccaggggcactggaggac

SEQ ID NO: 10560 - RNA, 20 nt, synthetic construct
  source 1..20: mol_type = other RNA
ggggggcccaggggcactgg

SEQ ID NO: 10561 - RNA, 20 nt, synthetic construct
  source 1..20: mol_type = other RNA
tcaggggggcccaggggcac

SEQ ID NO: 10562 - RNA, 20 nt, synthetic construct
  source 1..20: mol_type = other RNA
atgttctcaggggggcccag

SEQ ID NO: 10563 - RNA, 20 nt, synthetic construct
  source 1..20: mol_type = other RNA
aatgttctcaggggggccca

SEQ ID NO: 10564 - RNA, 20 nt, synthetic construct
  source 1..20: mol_type = other RNA
taatgttctcaggggggccc

SEQ ID NO: 10565 - RNA, 20 nt, synthetic construct
  source 1..20: mol_type = other RNA
ctgagaacattagtgctacg

SEQ ID NO: 10566 - RNA, 20 nt, synthetic construct
  source 1..20: mol_type = other RNA
gtagcactaatgttctcagg

SEQ ID NO: 10567 - RNA, 20 nt, synthetic construct
  source 1..20: mol_type = other RNA
cgtagcactaatgttctcag

SEQ ID NO: 10568 - RNA, 20 nt, synthetic construct
  source 1..20: mol_type = other RNA
gcgtagcactaatgttctca

SEQ ID NO: 10569 - RNA, 20 nt, synthetic construct
  source 1..20: mol_type = other RNA
cgcgtagcactaatgttctc

SEQ ID NO: 10570 - RNA, 20 nt, synthetic construct
  source 1..20: mol_type = other RNA
aacattagtgctacgcggaa

SEQ ID NO: 10571 - RNA, 20 nt, synthetic construct
  source 1..20: mol_type = other RNA
acattagtgctacgcggaat

SEQ ID NO: 10572 - RNA, 20 nt, synthetic construct
  source 1..20: mol_type = other RNA
tgctacgcggaatgggagcc

SEQ ID NO: 10573 - RNA, 20 nt, synthetic construct
  source 1..20: mol_type = other RNA
ggagccaggccttcgtgcat

SEQ ID NO: 10574 - RNA, 20 nt, synthetic construct
  source 1..20: mol_type = other RNA
cttgccaatgcacgaaggcc

SEQ ID NO: 10575 - RNA, 20 nt, synthetic construct
  source 1..20: mol_type = other RNA
tcgtgcattggcaagagccc

SEQ ID NO: 10576 - RNA, 20 nt, synthetic construct
  source 1..20: mol_type = other RNA
cgtgcattggcaagagcccc

SEQ ID NO: 10577 - RNA, 20 nt, synthetic construct
  source 1..20: mol_type = other RNA
gggctcttgccaatgcacga

SEQ ID NO: 10578 - RNA, 20 nt, synthetic construct
  source 1..20: mol_type = other RNA
agagccccgggcgcccctgc

SEQ ID NO: 10579 - RNA, 20 nt, synthetic construct
  source 1..20: mol_type = other RNA
gagccccgggcgcccctgca

SEQ ID NO: 10580 - RNA, 20 nt, synthetic construct
  source 1..20: mol_type = other RNA
gtaccctgcaggggcgcccg

SEQ ID NO: 10581 - RNA, 20 nt, synthetic construct
  source 1..20: mol_type = other RNA
ggtaccctgcaggggcgccc

SEQ ID NO: 10582 - RNA, 20 nt, synthetic construct
  source 1..20: mol_type = other RNA
gggtaccctgcaggggcgcc

SEQ ID NO: 10583 - RNA, 20 nt, synthetic construct
  source 1..20: mol_type = other RNA
cccctgcagggtaccctgtt

SEQ ID NO: 10584 - RNA, 20 nt, synthetic construct
  source 1..20: mol_type = other RNA
ccctgcagggtaccctgtta

SEQ ID NO: 10585 - RNA, 20 nt, synthetic construct
  source 1..20: mol_type = other RNA
cctaacagggtaccctgcag

SEQ ID NO: 10586 - RNA, 20 nt, synthetic construct
  source 1..20: mol_type = other RNA
ccctaacagggtaccctgca

SEQ ID NO: 10587 - RNA, 20 nt, synthetic construct
  source 1..20: mol_type = other RNA
agggtaccctgttagggtac

SEQ ID NO: 10588 - RNA, 20 nt, synthetic construct
  source 1..20: mol_type = other RNA
taccctgttagggtaccggc

SEQ ID NO: 10589 - RNA, 20 nt, synthetic construct
  source 1..20: mol_type = other RNA
cgccagccggtaccctaaca

SEQ ID NO: 10590 - RNA, 20 nt, synthetic construct
  source 1..20: mol_type = other RNA
acgccagccggtaccctaac

SEQ ID NO: 10591 - RNA, 20 nt, synthetic construct
  source 1..20: mol_type = other RNA
gggtaccggctggcgtatca

SEQ ID NO: 10592 - RNA, 20 nt, synthetic construct
  source 1..20: mol_type = other RNA
ccggctggcgtatcaaggcc

SEQ ID NO: 10593 - RNA, 20 nt, synthetic construct
  source 1..20: mol_type = other RNA
cctggccttgatacgccagc

SEQ ID NO: 10594 - RNA, 20 nt, synthetic construct
  source 1..20: mol_type = other RNA
tcaaggccaggacaccccag

SEQ ID NO: 10595 - RNA, 20 nt, synthetic construct
  source 1..20: mol_type = other RNA
aggccaggacaccccagagg

SEQ ID NO: 10596 - RNA, 20 nt, synthetic construct
  source 1..20: mol_type = other RNA
ggccaggacaccccagaggt

SEQ ID NO: 10597 - RNA, 20 nt, synthetic construct
  source 1..20: mol_type = other RNA
cacccacctctggggtgtcc

SEQ ID NO: 10598 - RNA, 20 nt, synthetic construct
  source 1..20: mol_type = other RNA
accccagaggtgggtgctgc

SEQ ID NO: 10599 - RNA, 20 nt, synthetic construct
  source 1..20: mol_type = other RNA
ccagaggtgggtgctgctgg

SEQ ID NO: 10600 - RNA, 20 nt, synthetic construct
  source 1..20: mol_type = other RNA
cagaggtgggtgctgctggt

SEQ ID NO: 10601 - RNA, 20 nt, synthetic construct
  source 1..20: mol_type = other RNA
accagcagcacccacctctg

SEQ ID NO: 10602 - RNA, 20 nt, synthetic construct
  source 1..20: mol_type = other RNA
caccagcagcacccacctct

SEQ ID NO: 10603 - RNA, 20 nt, synthetic construct
  source 1..20: mol_type = other RNA
ccaccagcagcacccacctc

SEQ ID NO: 10604 - RNA, 20 nt, synthetic construct
  source 1..20: mol_type = other RNA
gtgggtgctgctggtgggat

SEQ ID NO: 10605 - RNA, 20 nt, synthetic construct
  source 1..20: mol_type = other RNA
tgctgctggtgggattggag

SEQ ID NO: 10606 - RNA, 20 nt, synthetic construct
  source 1..20: mol_type = other RNA
ctggtgggattggagtggag

SEQ ID NO: 10607 - RNA, 20 nt, synthetic construct
  source 1..20: mol_type = other RNA
gggattggagtggagtggct

SEQ ID NO: 10608 - RNA, 20 nt, synthetic construct
  source 1..20: mol_type = other RNA
ggattggagtggagtggctt

SEQ ID NO: 10609 - RNA, 20 nt, synthetic construct
  source 1..20: mol_type = other RNA
gattggagtggagtggcttg

SEQ ID NO: 10610 - RNA, 20 nt, synthetic construct
  source 1..20: mol_type = other RNA
tggagtggagtggcttgggg

SEQ ID NO: 10611 - RNA, 20 nt, synthetic construct
  source 1..20: mol_type = other RNA
agtggagtggcttggggagg

SEQ ID NO: 10612 - RNA, 20 nt, synthetic construct
  source 1..20: mol_type = other RNA
gtggagtggcttggggagga

SEQ ID NO: 10613 - RNA, 20 nt, synthetic construct
  source 1..20: mol_type = other RNA
gagtggcttggggaggaggg

SEQ ID NO: 10614 - RNA, 20 nt, synthetic construct
  source 1..20: mol_type = other RNA
aggagggaggagaacatatc

SEQ ID NO: 10615 - RNA, 20 nt, synthetic construct
  source 1..20: mol_type = other RNA
ggagggaggagaacatatca

SEQ ID NO: 10616 - RNA, 20 nt, synthetic construct
  source 1..20: mol_type = other RNA
catatcagggcagacataga

SEQ ID NO: 10617 - RNA, 20 nt, synthetic construct
  source 1..20: mol_type = other RNA
gcagacatagatggttgtga

SEQ ID NO: 10618 - RNA, 20 nt, synthetic construct
  source 1..20: mol_type = other RNA
acatagatggttgtgaaggt

SEQ ID NO: 10619 - RNA, 20 nt, synthetic construct
  source 1..20: mol_type = other RNA
catagatggttgtgaaggtt

SEQ ID NO: 10620 - RNA, 20 nt, synthetic construct
  source 1..20: mol_type = other RNA
tacacaattgctctatgcct

SEQ ID NO: 10621 - RNA, 20 nt, synthetic construct
  source 1..20: mol_type = other RNA
acacaattgctctatgccta

SEQ ID NO: 10622 - RNA, 20 nt, synthetic construct
  source 1..20: mol_type = other RNA
cacaattgctctatgcctag

SEQ ID NO: 10623 - RNA, 20 nt, synthetic construct
  source 1..20: mol_type = other RNA
acaattgctctatgcctagg

SEQ ID NO: 10624 - RNA, 20 nt, synthetic construct
  source 1..20: mol_type = other RNA
ggatgaggagttggaggatg

SEQ ID NO: 10625 - RNA, 20 nt, synthetic construct
  source 1..20: mol_type = other RNA
agagcgttttgagaaagaga

SEQ ID NO: 10626 - RNA, 20 nt, synthetic construct
  source 1..20: mol_type = other RNA
gagcgttttgagaaagagat

SEQ ID NO: 10627 - RNA, 20 nt, synthetic construct
  source 1..20: mol_type = other RNA
agcgttttgagaaagagatg

SEQ ID NO: 10628 - RNA, 20 nt, synthetic construct
  source 1..20: mol_type = other RNA
ggcattgagcccgagagtga

SEQ ID NO: 10629 - RNA, 20 nt, synthetic construct
  source 1..20: mol_type = other RNA
gagagtgaaggcttaacagc

SEQ ID NO: 10630 - RNA, 20 nt, synthetic construct
  source 1..20: mol_type = other RNA
agagtgaaggcttaacagct

SEQ ID NO: 10631 - RNA, 20 nt, synthetic construct
  source 1..20: mol_type = other RNA
gctgttaagccttcactctc

SEQ ID NO: 10632 - RNA, 20 nt, synthetic construct
  source 1..20: mol_type = other RNA
agtgaaggcttaacagctgg

SEQ ID NO: 10633 - RNA, 20 nt, synthetic construct
  source 1..20: mol_type = other RNA
gtgaaggcttaacagctggg

SEQ ID NO: 10634 - RNA, 20 nt, synthetic construct
  source 1..20: mol_type = other RNA
ggcttaacagctggggggta

SEQ ID NO: 10635 - RNA, 20 nt, synthetic construct
  source 1..20: mol_type = other RNA
ttctaccctgatgccacttc

SEQ ID NO: 10636 - RNA, 20 nt, synthetic construct
  source 1..20: mol_type = other RNA
atgccacttctggacctcct

SEQ ID NO: 10637 - RNA, 20 nt, synthetic construct
  source 1..20: mol_type = other RNA
ggaggtccagaagtggcatc

SEQ ID NO: 10638 - RNA, 20 nt, synthetic construct
  source 1..20: mol_type = other RNA
gcacctaggaggtccagaag

SEQ ID NO: 10639 - RNA, 20 nt, synthetic construct
  source 1..20: mol_type = other RNA
ctggacctcctaggtgctaa

SEQ ID NO: 10640 - RNA, 20 nt, synthetic construct
  source 1..20: mol_type = other RNA
tcctaggtgctaatggacat

SEQ ID NO: 10641 - RNA, 20 nt, synthetic construct
  source 1..20: mol_type = other RNA
cctaggtgctaatggacata

SEQ ID NO: 10642 - RNA, 20 nt, synthetic construct
  source 1..20: mol_type = other RNA
tatgtccattagcacctagg

SEQ ID NO: 10643 - RNA, 20 nt, synthetic construct
  source 1..20: mol_type = other RNA
ccctatgtccattagcacct

SEQ ID NO: 10644 - RNA, 20 nt, synthetic construct
  source 1..20: mol_type = other RNA
tgctaatggacatagggcta

SEQ ID NO: 10645 - RNA, 20 nt, synthetic construct
  source 1..20: mol_type = other RNA
ggacatagggctaaggcaag

SEQ ID NO: 10646 - RNA, 20 nt, synthetic construct
  source 1..20: mol_type = other RNA
gctaaggcaagaggtgaccc

SEQ ID NO: 10647 - RNA, 20 nt, synthetic construct
  source 1..20: mol_type = other RNA
agaggtgaccctggagctgc

SEQ ID NO: 10648 - RNA, 20 nt, synthetic construct
  source 1..20: mol_type = other RNA
gaggtgaccctggagctgca

SEQ ID NO: 10649 - RNA, 20 nt, synthetic construct
  source 1..20: mol_type = other RNA
aggtgaccctggagctgcag

SEQ ID NO: 10650 - RNA, 20 nt, synthetic construct
  source 1..20: mol_type = other RNA
ggtgaccctggagctgcagg

SEQ ID NO: 10651 - RNA, 20 nt, synthetic construct
  source 1..20: mol_type = other RNA
accctggagctgcaggggga

SEQ ID NO: 10652 - RNA, 20 nt, synthetic construct
  source 1..20: mol_type = other RNA
ccctggagctgcagggggac

SEQ ID NO: 10653 - RNA, 20 nt, synthetic construct
  source 1..20: mol_type = other RNA
cccgtccccctgcagctcca

SEQ ID NO: 10654 - RNA, 20 nt, synthetic construct
  source 1..20: mol_type = other RNA
acccgtccccctgcagctcc

SEQ ID NO: 10655 - RNA, 20 nt, synthetic construct
  source 1..20: mol_type = other RNA
gtccaatctgacagtgtgtg

SEQ ID NO: 10656 - RNA, 20 nt, synthetic construct
  source 1..20: mol_type = other RNA
tgccacacacactgtcagat

SEQ ID NO: 10657 - RNA, 20 nt, synthetic construct
  source 1..20: mol_type = other RNA
gtggcagcctacactgctgc

SEQ ID NO: 10658 - RNA, 20 nt, synthetic construct
  source 1..20: mol_type = other RNA
tggcagcctacactgctgct

SEQ ID NO: 10659 - RNA, 20 nt, synthetic construct
  source 1..20: mol_type = other RNA
ggcagcctacactgctgctg

SEQ ID NO: 10660 - RNA, 20 nt, synthetic construct
  source 1..20: mol_type = other RNA
gcctacactgctgctgggga

SEQ ID NO: 10661 - RNA, 20 nt, synthetic construct
  source 1..20: mol_type = other RNA
tccatccccagcagcagtgt

SEQ ID NO: 10662 - RNA, 20 nt, synthetic construct
  source 1..20: mol_type = other RNA
ctgctgctggggatggaccc

SEQ ID NO: 10663 - RNA, 20 nt, synthetic construct
  source 1..20: mol_type = other RNA
ctggagcctcccagtacccc

SEQ ID NO: 10664 - RNA, 20 nt, synthetic construct
  source 1..20: mol_type = other RNA
gagcctcccagtacccctgg

SEQ ID NO: 10665 - RNA, 20 nt, synthetic construct
  source 1..20: mol_type = other RNA
caggggtactgggaggctcc

SEQ ID NO: 10666 - RNA, 20 nt, synthetic construct
  source 1..20: mol_type = other RNA
tcccagtacccctggaggcc

SEQ ID NO: 10667 - RNA, 20 nt, synthetic construct
  source 1..20: mol_type = other RNA
aggcctccaggggtactggg

SEQ ID NO: 10668 - RNA, 20 nt, synthetic construct
  source 1..20: mol_type = other RNA
gccaggcctccaggggtact

SEQ ID NO: 10669 - RNA, 20 nt, synthetic construct
  source 1..20: mol_type = other RNA
cgccaggcctccaggggtac

SEQ ID NO: 10670 - RNA, 20 nt, synthetic construct
  source 1..20: mol_type = other RNA
cccctggaggcctggcgccc

SEQ ID NO: 10671 - RNA, 20 nt, synthetic construct
  source 1..20: mol_type = other RNA
cctgggcgccaggcctccag

SEQ ID NO: 10672 - RNA, 20 nt, synthetic construct
  source 1..20: mol_type = other RNA
acctgggcgccaggcctcca

SEQ ID NO: 10673 - RNA, 20 nt, synthetic construct
  source 1..20: mol_type = other RNA
tacctgggcgccaggcctcc

SEQ ID NO: 10674 - RNA, 20 nt, synthetic construct
  source 1..20: mol_type = other RNA
tttggacttacctgggcgcc

SEQ ID NO: 10675 - RNA, 20 nt, synthetic construct
  source 1..20: mol_type = other RNA
gcatggctttggacttacct

SEQ ID NO: 10676 - RNA, 20 nt, synthetic construct
  source 1..20: mol_type = other RNA
ggcatggctttggacttacc

SEQ ID NO: 10677 - RNA, 20 nt, synthetic construct
  source 1..20: mol_type = other RNA
aagcaggttgggcatggctt

SEQ ID NO: 10678 - RNA, 20 nt, synthetic construct
  source 1..20: mol_type = other RNA
gggttgaagcaggttgggca

SEQ ID NO: 10679 - RNA, 20 nt, synthetic construct
  source 1..20: mol_type = other RNA
agacagggttgaagcaggtt

SEQ ID NO: 10680 - RNA, 20 nt, synthetic construct
  source 1..20: mol_type = other RNA
gagacagggttgaagcaggt

SEQ ID NO: 10681 - RNA, 20 nt, synthetic construct
  source 1..20: mol_type = other RNA
gggagagacagggttgaagc

SEQ ID NO: 10682 - RNA, 20 nt, synthetic construct
  source 1..20: mol_type = other RNA
agggctgtcagggagagaca

SEQ ID NO: 10683 - RNA, 20 nt, synthetic construct
  source 1..20: mol_type = other RNA
cagggctgtcagggagagac

SEQ ID NO: 10684 - RNA, 20 nt, synthetic construct
  source 1..20: mol_type = other RNA
ggagtaagtcagggctgtca

SEQ ID NO: 10685 - RNA, 20 nt, synthetic construct
  source 1..20: mol_type = other RNA
aggagtaagtcagggctgtc

SEQ ID NO: 10686 - RNA, 20 nt, synthetic construct
  source 1..20: mol_type = other RNA
aaggtacaaggagtaagtca

SEQ ID NO: 10687 - RNA, 20 nt, synthetic construct
  source 1..20: mol_type = other RNA
aaaggtacaaggagtaagtc

SEQ ID NO: 10688 - RNA, 20 nt, synthetic construct
  source 1..20: mol_type = other RNA
cggtaacactgaaaggtaca

SEQ ID NO: 10689 - RNA, 20 nt, synthetic construct
  source 1..20: mol_type = other RNA
tttcagtgttaccgcaactt

SEQ ID NO: 10690 - RNA, 20 nt, synthetic construct
  source 1..20: mol_type = other RNA
taagttgcggtaacactgaa

SEQ ID NO: 10691 - RNA, 20 nt, synthetic construct
  source 1..20: mol_type = other RNA
taggaacagggcctaagttg

SEQ ID NO: 10692 - RNA, 20 nt, synthetic construct
  source 1..20: mol_type = other RNA
taaggctcagggtaggaaca

SEQ ID NO: 10693 - RNA, 20 nt, synthetic construct
  source 1..20: mol_type = other RNA
gtaaggctcagggtaggaac

SEQ ID NO: 10694 - RNA, 20 nt, synthetic construct
  source 1..20: mol_type = other RNA
tggcacgagtaagggagtga

SEQ ID NO: 10695 - RNA, 20 nt, synthetic construct
  source 1..20: mol_type = other RNA
tgagggtgtggcacgagtaa

SEQ ID NO: 10696 - RNA, 20 nt, synthetic construct
  source 1..20: mol_type = other RNA
gtgagggtgtggcacgagta

SEQ ID NO: 10697 - RNA, 20 nt, synthetic construct
  source 1..20: mol_type = other RNA
cgggtaagggagtgagggtg

SEQ ID NO: 10698 - RNA, 20 nt, synthetic construct
  source 1..20: mol_type = other RNA
tggcacgggtaagggagtga

SEQ ID NO: 10699 - RNA, 20 nt, synthetic construct
  source 1..20: mol_type = other RNA
gtggcacgggtaagggagtg

SEQ ID NO: 10700 - RNA, 20 nt, synthetic construct
  source 1..20: mol_type = other RNA
taagggtgtggcacgggtaa

SEQ ID NO: 10701 - RNA, 20 nt, synthetic construct
  source 1..20: mol_type = other RNA
gtaagggtgtggcacgggta

SEQ ID NO: 10702 - RNA, 20 nt, synthetic construct
  source 1..20: mol_type = other RNA
agggagtaagggtgtggcac

SEQ ID NO: 10703 - RNA, 20 nt, synthetic construct
  source 1..20: mol_type = other RNA
aagggagtaagggtgtggca

SEQ ID NO: 10704 - RNA, 20 nt, synthetic construct
  source 1..20: mol_type = other RNA
cgggtaagggagtaagggtg

SEQ ID NO: 10705 - RNA, 20 nt, synthetic construct
  source 1..20: mol_type = other RNA
tggcacgggtaagggagtaa

SEQ ID NO: 10706 - RNA, 20 nt, synthetic construct
  source 1..20: mol_type = other RNA
gtggcacgggtaagggagta

SEQ ID NO: 10707 - RNA, 20 nt, synthetic construct
  source 1..20: mol_type = other RNA
gactggcgtggcacgggtaa

SEQ ID NO: 10708 - RNA, 20 nt, synthetic construct
  source 1..20: mol_type = other RNA
agactggcgtggcacgggta

SEQ ID NO: 10709 - RNA, 20 nt, synthetic construct
  source 1..20: mol_type = other RNA
ggacaagactggcgtggcac

SEQ ID NO: 10710 - RNA, 20 nt, synthetic construct
  source 1..20: mol_type = other RNA
aggacaagactggcgtggca

SEQ ID NO: 10711 - RNA, 20 nt, synthetic construct
  source 1..20: mol_type = other RNA
cagagaggacaagactggcg

SEQ ID NO: 10712 - RNA, 20 nt, synthetic construct
  source 1..20: mol_type = other RNA
gtgctcagagaggacaagac

SEQ ID NO: 10713 - RNA, 20 nt, synthetic construct
  source 1..20: mol_type = other RNA
gagaggagatgtgctcagag

SEQ ID NO: 10714 - RNA, 20 nt, synthetic construct
  source 1..20: mol_type = other RNA
tctctgtcctttcttctcac

SEQ ID NO: 10715 - RNA, 20 nt, synthetic construct
  source 1..20: mol_type = other RNA
ctctgtcctttcttctcaca

SEQ ID NO: 10716 - RNA, 20 nt, synthetic construct
  source 1..20: mol_type = other RNA
tgtgagaagaaaggacagag

SEQ ID NO: 10717 - RNA, 20 nt, synthetic construct
  source 1..20: mol_type = other RNA
tgcttgccctgtgagaagaa

SEQ ID NO: 10718 - RNA, 20 nt, synthetic construct
  source 1..20: mol_type = other RNA
agcacagccagtccaccagc

SEQ ID NO: 10719 - RNA, 20 nt, synthetic construct
  source 1..20: mol_type = other RNA
gcacagccagtccaccagct

SEQ ID NO: 10720 - RNA, 20 nt, synthetic construct
  source 1..20: mol_type = other RNA
gccagtccaccagctgggta

SEQ ID NO: 10721 - RNA, 20 nt, synthetic construct
  source 1..20: mol_type = other RNA
ccagtccaccagctgggtaa

SEQ ID NO: 10722 - RNA, 20 nt, synthetic construct
  source 1..20: mol_type = other RNA
cccttacccagctggtggac

SEQ ID NO: 10723 - RNA, 20 nt, synthetic construct
  source 1..20: mol_type = other RNA
ggaagcccttacccagctgg

SEQ ID NO: 10724 - RNA, 20 nt, synthetic construct
  source 1..20: mol_type = other RNA
tgtggaagcccttacccagc

SEQ ID NO: 10725 - RNA, 20 nt, synthetic construct
  source 1..20: mol_type = other RNA
gggaaggaggagatggggtg

SEQ ID NO: 10726 - RNA, 20 nt, synthetic construct
  source 1..20: mol_type = other RNA
gggtagggaaggaggagatg

SEQ ID NO: 10727 - RNA, 20 nt, synthetic construct
  source 1..20: mol_type = other RNA
agggtagggaaggaggagat

SEQ ID NO: 10728 - RNA, 20 nt, synthetic construct
  source 1..20: mol_type = other RNA
gagggtagggaaggaggaga

SEQ ID NO: 10729 - RNA, 20 nt, synthetic construct
  source 1..20: mol_type = other RNA
ggtgttgagggtagggaagg

SEQ ID NO: 10730 - RNA, 20 nt, synthetic construct
  source 1..20: mol_type = other RNA
tccctaccctcaacacctag

SEQ ID NO: 10731 - RNA, 20 nt, synthetic construct
  source 1..20: mol_type = other RNA
ccctaccctcaacacctagt

SEQ ID NO: 10732 - RNA, 20 nt, synthetic construct
  source 1..20: mol_type = other RNA
cctaccctcaacacctagtg

SEQ ID NO: 10733 - RNA, 20 nt, synthetic construct
  source 1..20: mol_type = other RNA
ctaccctcaacacctagtgg

SEQ ID NO: 10734 - RNA, 20 nt, synthetic construct
  source 1..20: mol_type = other RNA
cccactaggtgttgagggta

SEQ ID NO: 10735 - RNA, 20 nt, synthetic construct
  source 1..20: mol_type = other RNA
ccccactaggtgttgagggt

SEQ ID NO: 10736 - RNA, 20 nt, synthetic construct
  source 1..20: mol_type = other RNA
gtgcccccactaggtgttga

SEQ ID NO: 10737 - RNA, 20 nt, synthetic construct
  source 1..20: mol_type = other RNA
agtgcccccactaggtgttg

SEQ ID NO: 10738 - RNA, 20 nt, synthetic construct
  source 1..20: mol_type = other RNA
atggtgacagtgcccccact

SEQ ID NO: 10739 - RNA, 20 nt, synthetic construct
  source 1..20: mol_type = other RNA
ggatgtgcaatgagtatgca

SEQ ID NO: 10740 - RNA, 20 nt, synthetic construct
  source 1..20: mol_type = other RNA
tgagttagagaaacatgaaa

SEQ ID NO: 10741 - RNA, 20 nt, synthetic construct
  source 1..20: mol_type = other RNA
atgagttagagaaacatgaa

SEQ ID NO: 10742 - RNA, 20 nt, synthetic construct
  source 1..20: mol_type = other RNA
agatgtgcacatacttgatg

SEQ ID NO: 10743 - RNA, 20 nt, synthetic construct
  source 1..20: mol_type = other RNA
gtatgtgcacatctttgccg

SEQ ID NO: 10744 - RNA, 20 nt, synthetic construct
  source 1..20: mol_type = other RNA
gggagggaggcagaaggcct

SEQ ID NO: 10745 - RNA, 20 nt, synthetic construct
  source 1..20: mol_type = other RNA
tgatgtgggagggaggcaga

SEQ ID NO: 10746 - RNA, 20 nt, synthetic construct
  source 1..20: mol_type = other RNA
tccctcccacatcacccctt

SEQ ID NO: 10747 - RNA, 20 nt, synthetic construct
  source 1..20: mol_type = other RNA
ccctcccacatcaccccttt

SEQ ID NO: 10748 - RNA, 20 nt, synthetic construct
  source 1..20: mol_type = other RNA
aaaggggtgatgtgggaggg

SEQ ID NO: 10749 - RNA, 20 nt, synthetic construct
  source 1..20: mol_type = other RNA
cccaaaggggtgatgtggga

SEQ ID NO: 10750 - RNA, 20 nt, synthetic construct
  source 1..20: mol_type = other RNA
acccaaaggggtgatgtggg

SEQ ID NO: 10751 - RNA, 20 nt, synthetic construct
  source 1..20: mol_type = other RNA
gggacccaaaggggtgatgt

SEQ ID NO: 10752 - RNA, 20 nt, synthetic construct
  source 1..20: mol_type = other RNA
tgggacccaaaggggtgatg

SEQ ID NO: 10753 - RNA, 20 nt, synthetic construct
  source 1..20: mol_type = other RNA
ccctttgggtcccagagagc

SEQ ID NO: 10754 - RNA, 20 nt, synthetic construct
  source 1..20: mol_type = other RNA
cagctctctgggacccaaag

SEQ ID NO: 10755 - RNA, 20 nt, synthetic construct
  source 1..20: mol_type = other RNA
ccagctctctgggacccaaa

SEQ ID NO: 10756 - RNA, 20 nt, synthetic construct
  source 1..20: mol_type = other RNA
tccagctctctgggacccaa

SEQ ID NO: 10757 - RNA, 20 nt, synthetic construct
  source 1..20: mol_type = other RNA
gtcccagagagctggatcca

SEQ ID NO: 10758 - RNA, 20 nt, synthetic construct
  source 1..20: mol_type = other RNA
agccttggatccagctctct

SEQ ID NO: 10759 - RNA, 20 nt, synthetic construct
  source 1..20: mol_type = other RNA
aagccttggatccagctctc

SEQ ID NO: 10760 - RNA, 20 nt, synthetic construct
  source 1..20: mol_type = other RNA
acaggtcatggatgaagcct

SEQ ID NO: 10761 - RNA, 20 nt, synthetic construct
  source 1..20: mol_type = other RNA
ggggtatgaggaacaggtca

SEQ ID NO: 10762 - RNA, 20 nt, synthetic construct
  source 1..20: mol_type = other RNA
tatcagggggtatgaggaac

SEQ ID NO: 10763 - RNA, 20 nt, synthetic construct
  source 1..20: mol_type = other RNA
ctcataccccctgatagtga

SEQ ID NO: 10764 - RNA, 20 nt, synthetic construct
  source 1..20: mol_type = other RNA
cttcactatcagggggtatg

SEQ ID NO: 10765 - RNA, 20 nt, synthetic construct
  source 1..20: mol_type = other RNA
aaggttccttcactatcagg

SEQ ID NO: 10766 - RNA, 20 nt, synthetic construct
  source 1..20: mol_type = other RNA
gaaggttccttcactatcag

SEQ ID NO: 10767 - RNA, 20 nt, synthetic construct
  source 1..20: mol_type = other RNA
tgaaggttccttcactatca

SEQ ID NO: 10768 - RNA, 20 nt, synthetic construct
  source 1..20: mol_type = other RNA
ttgaaggttccttcactatc

SEQ ID NO: 10769 - RNA, 20 nt, synthetic construct
  source 1..20: mol_type = other RNA
cttcaactcctgccttctcg

SEQ ID NO: 10770 - RNA, 20 nt, synthetic construct
  source 1..20: mol_type = other RNA
cacgagaaggcaggagttga

SEQ ID NO: 10771 - RNA, 20 nt, synthetic construct
  source 1..20: mol_type = other RNA
ctcctgccttctcgtggccc

SEQ ID NO: 10772 - RNA, 20 nt, synthetic construct
  source 1..20: mol_type = other RNA
ctgccttctcgtggccctgg

SEQ ID NO: 10773 - RNA, 20 nt, synthetic construct
  source 1..20: mol_type = other RNA
caccagggccacgagaaggc

SEQ ID NO: 10774 - RNA, 20 nt, synthetic construct
  source 1..20: mol_type = other RNA
ataccaccagggccacgaga

SEQ ID NO: 10775 - RNA, 20 nt, synthetic construct
  source 1..20: mol_type = other RNA
ccctggtggtatgtactgct

SEQ ID NO: 10776 - RNA, 20 nt, synthetic construct
  source 1..20: mol_type = other RNA
cctagcagtacataccacca

SEQ ID NO: 10777 - RNA, 20 nt, synthetic construct
  source 1..20: mol_type = other RNA
tcctagcagtacataccacc

SEQ ID NO: 10778 - RNA, 20 nt, synthetic construct
  source 1..20: mol_type = other RNA
tgtactgctaggagcagtcg

SEQ ID NO: 10779 - RNA, 20 nt, synthetic construct
  source 1..20: mol_type = other RNA
cgctgcctgtgtcctcatct

SEQ ID NO: 10780 - RNA, 20 nt, synthetic construct
  source 1..20: mol_type = other RNA
caagatgaggacacaggcag

SEQ ID NO: 10781 - RNA, 20 nt, synthetic construct
  source 1..20: mol_type = other RNA
gagagccaagatgaggacac

SEQ ID NO: 10782 - RNA, 20 nt, synthetic construct
  source 1..20: mol_type = other RNA
caaggaagagagccaagatg

SEQ ID NO: 10783 - RNA, 20 nt, synthetic construct
  source 1..20: mol_type = other RNA
tggctctcttccttgtccac

SEQ ID NO: 10784 - RNA, 20 nt, synthetic construct
  source 1..20: mol_type = other RNA
ccttgtccaccggcgaaaga

SEQ ID NO: 10785 - RNA, 20 nt, synthetic construct
  source 1..20: mol_type = other RNA
ccttctttcgccggtggaca

SEQ ID NO: 10786 - RNA, 20 nt, synthetic construct
  source 1..20: mol_type = other RNA
gggtctccttctttcgccgg

SEQ ID NO: 10787 - RNA, 20 nt, synthetic construct
  source 1..20: mol_type = other RNA
cgaaagaaggagacccgtta

SEQ ID NO: 10788 - RNA, 20 nt, synthetic construct
  source 1..20: mol_type = other RNA
gaaagaaggagacccgttat

SEQ ID NO: 10789 - RNA, 20 nt, synthetic construct
  source 1..20: mol_type = other RNA
gagacccgttatgggtgagt

SEQ ID NO: 10790 - RNA, 20 nt, synthetic construct
  source 1..20: mol_type = other RNA
ggttccaactcacccataac

SEQ ID NO: 10791 - RNA, 20 nt, synthetic construct
  source 1..20: mol_type = other RNA
atgggtgagttggaaccaca

SEQ ID NO: 10792 - RNA, 20 nt, synthetic construct
  source 1..20: mol_type = other RNA
tgggtgagttggaaccacat

SEQ ID NO: 10793 - RNA, 20 nt, synthetic construct
  source 1..20: mol_type = other RNA
gggtgagttggaaccacatg

SEQ ID NO: 10794 - RNA, 20 nt, synthetic construct
  source 1..20: mol_type = other RNA
tgagttggaaccacatgggg

SEQ ID NO: 10795 - RNA, 20 nt, synthetic construct
  source 1..20: mol_type = other RNA
aaccacatggggaggctgtg

SEQ ID NO: 10796 - RNA, 20 nt, synthetic construct
  source 1..20: mol_type = other RNA
catggggaggctgtgtggcc

SEQ ID NO: 10797 - RNA, 20 nt, synthetic construct
  source 1..20: mol_type = other RNA
atggggaggctgtgtggcct

SEQ ID NO: 10798 - RNA, 20 nt, synthetic construct
  source 1..20: mol_type = other RNA
ggccacacagcctccccatg

SEQ ID NO: 10799 - RNA, 20 nt, synthetic construct
  source 1..20: mol_type = other RNA
ggaggctgtgtggcctggga

SEQ ID NO: 10800 - RNA, 20 nt, synthetic construct
  source 1..20: mol_type = other RNA
ctgtgtggcctgggatggag

SEQ ID NO: 10801 - RNA, 20 nt, synthetic construct
  source 1..20: mol_type = other RNA
gtggcctgggatggagaggc

SEQ ID NO: 10802 - RNA, 20 nt, synthetic construct
  source 1..20: mol_type = other RNA
gcctgggatggagaggctgg

SEQ ID NO: 10803 - RNA, 20 nt, synthetic construct
  source 1..20: mol_type = other RNA
gggatggagaggctggaggc

SEQ ID NO: 10804 - RNA, 20 nt, synthetic construct
  source 1..20: mol_type = other RNA
ggatggagaggctggaggca

SEQ ID NO: 10805 - RNA, 20 nt, synthetic construct
  source 1..20: mol_type = other RNA
gcctccagcctctccatccc

SEQ ID NO: 10806 - RNA, 20 nt, synthetic construct
  source 1..20: mol_type = other RNA
tggagaggctggaggcaggg

SEQ ID NO: 10807 - RNA, 20 nt, synthetic construct
  source 1..20: mol_type = other RNA
tggaggcagggaggccagtg

SEQ ID NO: 10808 - RNA, 20 nt, synthetic construct
  source 1..20: mol_type = other RNA
aggcagggaggccagtgagg

SEQ ID NO: 10809 - RNA, 20 nt, synthetic construct
  source 1..20: mol_type = other RNA
agggaggccagtgaggaggc

SEQ ID NO: 10810 - RNA, 20 nt, synthetic construct
  source 1..20: mol_type = other RNA
gccagtgaggaggctggtgc

SEQ ID NO: 10811 - RNA, 20 nt, synthetic construct
  source 1..20: mol_type = other RNA
agtgaggaggctggtgcagg

SEQ ID NO: 10812 - RNA, 20 nt, synthetic construct
  source 1..20: mol_type = other RNA
tcctgcaccagcctcctcac

SEQ ID NO: 10813 - RNA, 20 nt, synthetic construct
  source 1..20: mol_type = other RNA
gatgactaagaatcagaatg

SEQ ID NO: 10814 - RNA, 20 nt, synthetic construct
  source 1..20: mol_type = other RNA
atgactaagaatcagaatga

SEQ ID NO: 10815 - RNA, 20 nt, synthetic construct
  source 1..20: mol_type = other RNA
taagaatcagaatgagggca

SEQ ID NO: 10816 - RNA, 20 nt, synthetic construct
  source 1..20: mol_type = other RNA
aagaatcagaatgagggcaa

SEQ ID NO: 10817 - RNA, 20 nt, synthetic construct
  source 1..20: mol_type = other RNA
caaatgttagcacagagggc

SEQ ID NO: 10818 - RNA, 20 nt, synthetic construct
  source 1..20: mol_type = other RNA
tgttagcacagagggcaggc

SEQ ID NO: 10819 - RNA, 20 nt, synthetic construct
  source 1..20: mol_type = other RNA
gttagcacagagggcaggca

SEQ ID NO: 10820 - RNA, 20 nt, synthetic construct
  source 1..20: mol_type = other RNA
cagagggcaggcagggcttg

SEQ ID NO: 10821 - RNA, 20 nt, synthetic construct
  source 1..20: mol_type = other RNA
ggcagggcttgaggctgaga

SEQ ID NO: 10822 - RNA, 20 nt, synthetic construct
  source 1..20: mol_type = other RNA
gatggtgcttgctcaactgc

SEQ ID NO: 10823 - RNA, 20 nt, synthetic construct
  source 1..20: mol_type = other RNA
tgctcaactgctggttgagt

SEQ ID NO: 10824 - RNA, 20 nt, synthetic construct
  source 1..20: mol_type = other RNA
gctcaactgctggttgagta

SEQ ID NO: 10825 - RNA, 20 nt, synthetic construct
  source 1..20: mol_type = other RNA
ctcaactgctggttgagtag

SEQ ID NO: 10826 - RNA, 20 nt, synthetic construct
  source 1..20: mol_type = other RNA
tcaactgctggttgagtagg

SEQ ID NO: 10827 - RNA, 20 nt, synthetic construct
  source 1..20: mol_type = other RNA
gttgagtagggggttccaca

SEQ ID NO: 10828 - RNA, 20 nt, synthetic construct
  source 1..20: mol_type = other RNA
gagggcagggaaaaaccatg

SEQ ID NO: 10829 - RNA, 20 nt, synthetic construct
  source 1..20: mol_type = other RNA
agggggagtaggtgagggca

SEQ ID NO: 10830 - RNA, 20 nt, synthetic construct
  source 1..20: mol_type = other RNA
gagggggagtaggtgagggc

SEQ ID NO: 10831 - RNA, 20 nt, synthetic construct
  source 1..20: mol_type = other RNA
gggggagggggagtaggtga

SEQ ID NO: 10832 - RNA, 20 nt, synthetic construct
  source 1..20: mol_type = other RNA
ggggggagggggagtaggtg

SEQ ID NO: 10833 - RNA, 20 nt, synthetic construct
  source 1..20: mol_type = other RNA
ctctgggggggagggggagt

SEQ ID NO: 10834 - RNA, 20 nt, synthetic construct
  source 1..20: mol_type = other RNA
acacttctctgggggggagg

SEQ ID NO: 10835 - RNA, 20 nt, synthetic construct
  source 1..20: mol_type = other RNA
aacacttctctgggggggag

SEQ ID NO: 10836 - RNA, 20 nt, synthetic construct
  source 1..20: mol_type = other RNA
aaacacttctctggggggga

SEQ ID NO: 10837 - RNA, 20 nt, synthetic construct
  source 1..20: mol_type = other RNA
caaacacttctctggggggg

SEQ ID NO: 10838 - RNA, 20 nt, synthetic construct
  source 1..20: mol_type = other RNA
gttcaaacacttctctgggg

SEQ ID NO: 10839 - RNA, 20 nt, synthetic construct
  source 1..20: mol_type = other RNA
ggttcaaacacttctctggg

SEQ ID NO: 10840 - RNA, 20 nt, synthetic construct
  source 1..20: mol_type = other RNA
tggttcaaacacttctctgg

SEQ ID NO: 10841 - RNA, 20 nt, synthetic construct
  source 1..20: mol_type = other RNA
ttggttcaaacacttctctg

SEQ ID NO: 10842 - RNA, 20 nt, synthetic construct
  source 1..20: mol_type = other RNA
gttggttcaaacacttctct

SEQ ID NO: 10843 - RNA, 20 nt, synthetic construct
  source 1..20: mol_type = other RNA
tgttggttcaaacacttctc

SEQ ID NO: 10844 - RNA, 20 nt, synthetic construct
  source 1..20: mol_type = other RNA
tttgaaccaacagtggaaag

SEQ ID NO: 10845 - RNA, 20 nt, synthetic construct
  source 1..20: mol_type = other RNA
aacagtggaaagaggtgaac

SEQ ID NO: 10846 - RNA, 20 nt, synthetic construct
  source 1..20: mol_type = other RNA
agttcacctctttccactgt

SEQ ID NO: 10847 - RNA, 20 nt, synthetic construct
  source 1..20: mol_type = other RNA
aaagaggtgaactggtagtc

SEQ ID NO: 10848 - RNA, 20 nt, synthetic construct
  source 1..20: mol_type = other RNA
tgcgcaagtcctacagtcgt

SEQ ID NO: 10849 - RNA, 20 nt, synthetic construct
  source 1..20: mol_type = other RNA
ttcagtggtccgacgactgt

SEQ ID NO: 10850 - RNA, 20 nt, synthetic construct
  source 1..20: mol_type = other RNA
tcacttacaggtagcttcag

SEQ ID NO: 10851 - RNA, 20 nt, synthetic construct
  source 1..20: mol_type = other RNA
ggggcatagggttcacttac

SEQ ID NO: 10852 - RNA, 20 nt, synthetic construct
  source 1..20: mol_type = other RNA
aaccctatgccccactgccc

SEQ ID NO: 10853 - RNA, 20 nt, synthetic construct
  source 1..20: mol_type = other RNA
tatgccccactgccctggcc

SEQ ID NO: 10854 - RNA, 20 nt, synthetic construct
  source 1..20: mol_type = other RNA
ggccagggcagtggggcata

SEQ ID NO: 10855 - RNA, 20 nt, synthetic construct
  source 1..20: mol_type = other RNA
aggccagggcagtggggcat

SEQ ID NO: 10856 - RNA, 20 nt, synthetic construct
  source 1..20: mol_type = other RNA
agatccaggccagggcagtg

SEQ ID NO: 10857 - RNA, 20 nt, synthetic construct
  source 1..20: mol_type = other RNA
tagatccaggccagggcagt

SEQ ID NO: 10858 - RNA, 20 nt, synthetic construct
  source 1..20: mol_type = other RNA
ttagatccaggccagggcag

SEQ ID NO: 10859 - RNA, 20 nt, synthetic construct
  source 1..20: mol_type = other RNA
cagcctttagatccaggcca

SEQ ID NO: 10860 - RNA, 20 nt, synthetic construct
  source 1..20: mol_type = other RNA
acagcctttagatccaggcc

SEQ ID NO: 10861 - RNA, 20 nt, synthetic construct
  source 1..20: mol_type = other RNA
tctctacagcctttagatcc

SEQ ID NO: 10862 - RNA, 20 nt, synthetic construct
  source 1..20: mol_type = other RNA
tctaaaggctgtagagaatc

SEQ ID NO: 10863 - RNA, 20 nt, synthetic construct
  source 1..20: mol_type = other RNA
ctgtagagaatctggcctgc

SEQ ID NO: 10864 - RNA, 20 nt, synthetic construct
  source 1..20: mol_type = other RNA
tgtagagaatctggcctgct

SEQ ID NO: 10865 - RNA, 20 nt, synthetic construct
  source 1..20: mol_type = other RNA
cacatgtacagaagcccagc

SEQ ID NO: 10866 - RNA, 20 nt, synthetic construct
  source 1..20: mol_type = other RNA
tgtgagccaaaagtttctaa

SEQ ID NO: 10867 - RNA, 20 nt, synthetic construct
  source 1..20: mol_type = other RNA
ccaaaagtttctaaaggcct

SEQ ID NO: 10868 - RNA, 20 nt, synthetic construct
  source 1..20: mol_type = other RNA
caaaagtttctaaaggcctt

SEQ ID NO: 10869 - RNA, 20 nt, synthetic construct
  source 1..20: mol_type = other RNA
ccaaggcctttagaaacttt

SEQ ID NO: 10870 - RNA, 20 nt, synthetic construct
  source 1..20: mol_type = other RNA
gtatgtcagtgtttcaacaa

SEQ ID NO: 10871 - RNA, 20 nt, synthetic construct
  source 1..20: mol_type = other RNA
aacaatggatctatccctac

SEQ ID NO: 10872 - RNA, 20 nt, synthetic construct
  source 1..20: mol_type = other RNA
aatggatctatccctactgg

SEQ ID NO: 10873 - RNA, 20 nt, synthetic construct
  source 1..20: mol_type = other RNA
atggatctatccctactggt

SEQ ID NO: 10874 - RNA, 20 nt, synthetic construct
  source 1..20: mol_type = other RNA
gtgacattcacccaccagta

SEQ ID NO: 10875 - RNA, 20 nt, synthetic construct
  source 1..20: mol_type = other RNA
ggtgacattcacccaccagt

SEQ ID NO: 10876 - RNA, 20 nt, synthetic construct
  source 1..20: mol_type = other RNA
atggagcagggctgacattc

SEQ ID NO: 10877 - RNA, 20 nt, synthetic construct
  source 1..20: mol_type = other RNA
gtggacagagtcatggagca

SEQ ID NO: 10878 - RNA, 20 nt, synthetic construct
  source 1..20: mol_type = other RNA
ggtggacagagtcatggagc

SEQ ID NO: 10879 - RNA, 20 nt, synthetic construct
  source 1..20: mol_type = other RNA
ggttggggtggacagagtca

SEQ ID NO: 10880 - RNA, 20 nt, synthetic construct
  source 1..20: mol_type = other RNA
cactgcatgcaaggttgggg

SEQ ID NO: 10881 - RNA, 20 nt, synthetic construct
  source 1..20: mol_type = other RNA
gttcactgcatgcaaggttg

SEQ ID NO: 10882 - RNA, 20 nt, synthetic construct
  source 1..20: mol_type = other RNA
tgttcactgcatgcaaggtt

SEQ ID NO: 10883 - RNA, 20 nt, synthetic construct
  source 1..20: mol_type = other RNA
cttgcatgcagtgaacagcc

SEQ ID NO: 10884 - RNA, 20 nt, synthetic construct
  source 1..20: mol_type = other RNA
ttgcatgcagtgaacagcct

SEQ ID NO: 10885 - RNA, 20 nt, synthetic construct
  source 1..20: mol_type = other RNA
caggctgttcactgcatgca

SEQ ID NO: 10886 - RNA, 20 nt, synthetic construct
  source 1..20: mol_type = other RNA
gggcatcagtgaagagctga

SEQ ID NO: 10887 - RNA, 20 nt, synthetic construct
  source 1..20: mol_type = other RNA
tcagctcttcactgatgccc

SEQ ID NO: 10888 - RNA, 20 nt, synthetic construct
  source 1..20: mol_type = other RNA
aagagctgaaggagaagctg

SEQ ID NO: 10889 - RNA, 20 nt, synthetic construct
  source 1..20: mol_type = other RNA
agagctgaaggagaagctgc

SEQ ID NO: 10890 - RNA, 20 nt, synthetic construct
  source 1..20: mol_type = other RNA
ggagaagctgcgggatgtga

SEQ ID NO: 10891 - RNA, 20 nt, synthetic construct
  source 1..20: mol_type = other RNA
gaagctgcgggatgtgatgg

SEQ ID NO: 10892 - RNA, 20 nt, synthetic construct
  source 1..20: mol_type = other RNA
tgcgggatgtgatggtggac

SEQ ID NO: 10893 - RNA, 20 nt, synthetic construct
  source 1..20: mol_type = other RNA
tgtgatggtggaccggcaca

SEQ ID NO: 10894 - RNA, 20 nt, synthetic construct
  source 1..20: mol_type = other RNA
gatggtggaccggcacaagg

SEQ ID NO: 10895 - RNA, 20 nt, synthetic construct
  source 1..20: mol_type = other RNA
ggaccggcacaaggtggccc

SEQ ID NO: 10896 - RNA, 20 nt, synthetic construct
  source 1..20: mol_type = other RNA
gaccggcacaaggtggccct

SEQ ID NO: 10897 - RNA, 20 nt, synthetic construct
  source 1..20: mol_type = other RNA
accggcacaaggtggccctg

SEQ ID NO: 10898 - RNA, 20 nt, synthetic construct
  source 1..20: mol_type = other RNA
tccccagggccaccttgtgc

SEQ ID NO: 10899 - RNA, 20 nt, synthetic construct
  source 1..20: mol_type = other RNA
ggtggccctggggaagactc

SEQ ID NO: 10900 - RNA, 20 nt, synthetic construct
  source 1..20: mol_type = other RNA
gtggccctggggaagactct

SEQ ID NO: 10901 - RNA, 20 nt, synthetic construct
  source 1..20: mol_type = other RNA
cctggggaagactctgggag

SEQ ID NO: 10902 - RNA, 20 nt, synthetic construct
  source 1..20: mol_type = other RNA
ctggggaagactctgggaga

SEQ ID NO: 10903 - RNA, 20 nt, synthetic construct
  source 1..20: mol_type = other RNA
ctctcccagagtcttcccca

SEQ ID NO: 10904 - RNA, 20 nt, synthetic construct
  source 1..20: mol_type = other RNA
cctctcccagagtcttcccc

SEQ ID NO: 10905 - RNA, 20 nt, synthetic construct
  source 1..20: mol_type = other RNA
ctgggagagggtgagtcccc

SEQ ID NO: 10906 - RNA, 20 nt, synthetic construct
  source 1..20: mol_type = other RNA
ggatgtgtgtatgctgccgg

SEQ ID NO: 10907 - RNA, 20 nt, synthetic construct
  source 1..20: mol_type = other RNA
aggatgtgtgtatgctgccg

SEQ ID NO: 10908 - RNA, 20 nt, synthetic construct
  source 1..20: mol_type = other RNA
aaggatgtgtgtatgctgcc

SEQ ID NO: 10909 - RNA, 20 nt, synthetic construct
  source 1..20: mol_type = other RNA
gaaggatgtgtgtatgctgc

SEQ ID NO: 10910 - RNA, 20 nt, synthetic construct
  source 1..20: mol_type = other RNA
caggatctcagaagttcaga

SEQ ID NO: 10911 - RNA, 20 nt, synthetic construct
  source 1..20: mol_type = other RNA
gggtgggagtgtggaagtgc

SEQ ID NO: 10912 - RNA, 20 nt, synthetic construct
  source 1..20: mol_type = other RNA
ccacactcccacccaactat

SEQ ID NO: 10913 - RNA, 20 nt, synthetic construct
  source 1..20: mol_type = other RNA
cctatagttgggtgggagtg

SEQ ID NO: 10914 - RNA, 20 nt, synthetic construct
  source 1..20: mol_type = other RNA
tgtatttcctatagttgggt

SEQ ID NO: 10915 - RNA, 20 nt, synthetic construct
  source 1..20: mol_type = other RNA
ctgtatttcctatagttggg

SEQ ID NO: 10916 - RNA, 20 nt, synthetic construct
  source 1..20: mol_type = other RNA
ggactgtatttcctatagtt

SEQ ID NO: 10917 - RNA, 20 nt, synthetic construct
  source 1..20: mol_type = other RNA
tataggaaatacagtcccca

SEQ ID NO: 10918 - RNA, 20 nt, synthetic construct
  source 1..20: mol_type = other RNA
ataggaaatacagtccccac

SEQ ID NO: 10919 - RNA, 20 nt, synthetic construct
  source 1..20: mol_type = other RNA
cagtccccacgggccctctg

SEQ ID NO: 10920 - RNA, 20 nt, synthetic construct
  source 1..20: mol_type = other RNA
ctgacctcagagggcccgtg

SEQ ID NO: 10921 - RNA, 20 nt, synthetic construct
  source 1..20: mol_type = other RNA
actgacctcagagggcccgt

SEQ ID NO: 10922 - RNA, 20 nt, synthetic construct
  source 1..20: mol_type = other RNA
cactgacctcagagggcccg

SEQ ID NO: 10923 - RNA, 20 nt, synthetic construct
  source 1..20: mol_type = other RNA
ctgaggtcagtgtctccctc

SEQ ID NO: 10924 - RNA, 20 nt, synthetic construct
  source 1..20: mol_type = other RNA
agggagacactgacctcaga

SEQ ID NO: 10925 - RNA, 20 nt, synthetic construct
  source 1..20: mol_type = other RNA
gagggagacactgacctcag

SEQ ID NO: 10926 - RNA, 20 nt, synthetic construct
  source 1..20: mol_type = other RNA
gtctccctctggccccccac

SEQ ID NO: 10927 - RNA, 20 nt, synthetic construct
  source 1..20: mol_type = other RNA
tggccccccacaggagagtt

SEQ ID NO: 10928 - RNA, 20 nt, synthetic construct
  source 1..20: mol_type = other RNA
actctcctgtggggggccag

SEQ ID NO: 10929 - RNA, 20 nt, synthetic construct
  source 1..20: mol_type = other RNA
gctccaaactctcctgtggg

SEQ ID NO: 10930 - RNA, 20 nt, synthetic construct
  source 1..20: mol_type = other RNA
agctccaaactctcctgtgg

SEQ ID NO: 10931 - RNA, 20 nt, synthetic construct
  source 1..20: mol_type = other RNA
cagctccaaactctcctgtg

SEQ ID NO: 10932 - RNA, 20 nt, synthetic construct
  source 1..20: mol_type = other RNA
acagctccaaactctcctgt

SEQ ID NO: 10933 - RNA, 20 nt, synthetic construct
  source 1..20: mol_type = other RNA
cacagctccaaactctcctg

SEQ ID NO: 10934 - RNA, 20 nt, synthetic construct
  source 1..20: mol_type = other RNA
gagtttggagctgtgatgga

SEQ ID NO: 10935 - RNA, 20 nt, synthetic construct
  source 1..20: mol_type = other RNA
gatggaaggccagctcaacc

SEQ ID NO: 10936 - RNA, 20 nt, synthetic construct
  source 1..20: mol_type = other RNA
tggagtcgtcctggttgagc

SEQ ID NO: 10937 - RNA, 20 nt, synthetic construct
  source 1..20: mol_type = other RNA
ccaggacgactccatcctca

SEQ ID NO: 10938 - RNA, 20 nt, synthetic construct
  source 1..20: mol_type = other RNA
ggacgactccatcctcaagg

SEQ ID NO: 10939 - RNA, 20 nt, synthetic construct
  source 1..20: mol_type = other RNA
ccttgaggatggagtcgtcc

SEQ ID NO: 10940 - RNA, 20 nt, synthetic construct
  source 1..20: mol_type = other RNA
cttcacagccaccttgagga

SEQ ID NO: 10941 - RNA, 20 nt, synthetic construct
  source 1..20: mol_type = other RNA
tcgtcttcacagccaccttg

SEQ ID NO: 10942 - RNA, 20 nt, synthetic construct
  source 1..20: mol_type = other RNA
tgagttacgtgcacatgtgt

SEQ ID NO: 10943 - RNA, 20 nt, synthetic construct
  source 1..20: mol_type = other RNA
gggcatagggaaggagctgg

SEQ ID NO: 10944 - RNA, 20 nt, synthetic construct
  source 1..20: mol_type = other RNA
ggggcatagggaaggagctg

SEQ ID NO: 10945 - RNA, 20 nt, synthetic construct
  source 1..20: mol_type = other RNA
aggggcatagggaaggagct

SEQ ID NO: 10946 - RNA, 20 nt, synthetic construct
  source 1..20: mol_type = other RNA
caggggcatagggaaggagc

SEQ ID NO: 10947 - RNA, 20 nt, synthetic construct
  source 1..20: mol_type = other RNA
ctgtctcaggggcataggga

SEQ ID NO: 10948 - RNA, 20 nt, synthetic construct
  source 1..20: mol_type = other RNA
tcttctgtctcaggggcata

SEQ ID NO: 10949 - RNA, 20 nt, synthetic construct
  source 1..20: mol_type = other RNA
ctcttctgtctcaggggcat

SEQ ID NO: 10950 - RNA, 20 nt, synthetic construct
  source 1..20: mol_type = other RNA
cttgctctcttctgtctcag

SEQ ID NO: 10951 - RNA, 20 nt, synthetic construct
  source 1..20: mol_type = other RNA
gcttgctctcttctgtctca

SEQ ID NO: 10952 - RNA, 20 nt, synthetic construct
  source 1..20: mol_type = other RNA
tgcttgctctcttctgtctc

SEQ ID NO: 10953 - RNA, 20 nt, synthetic construct
  source 1..20: mol_type = other RNA
tagccatagcttagaacttc

SEQ ID NO: 10954 - RNA, 20 nt, synthetic construct
  source 1..20: mol_type = other RNA
acaccagaagttctaagcta

SEQ ID NO: 10955 - RNA, 20 nt, synthetic construct
  source 1..20: mol_type = other RNA
aacttctggtgtttccagat

SEQ ID NO: 10956 - RNA, 20 nt, synthetic construct
  source 1..20: mol_type = other RNA
tggtgtttccagataggcaa

SEQ ID NO: 10957 - RNA, 20 nt, synthetic construct
  source 1..20: mol_type = other RNA
gatgatgatgatgatgatga

SEQ ID NO: 10958 - RNA, 20 nt, synthetic construct
  source 1..20: mol_type = other RNA
tgatgatgatgatgatggag

SEQ ID NO: 10959 - RNA, 20 nt, synthetic construct
  source 1..20: mol_type = other RNA
tgatgatgatgatggagtgg

SEQ ID NO: 10960 - RNA, 20 nt, synthetic construct
  source 1..20: mol_type = other RNA
tgatgatgatggagtggagg

SEQ ID NO: 10961 - RNA, 20 nt, synthetic construct
  source 1..20: mol_type = other RNA
tgatgatggagtggaggtgg

SEQ ID NO: 10962 - RNA, 20 nt, synthetic construct
  source 1..20: mol_type = other RNA
gatgatggagtggaggtgga

SEQ ID NO: 10963 - RNA, 20 nt, synthetic construct
  source 1..20: mol_type = other RNA
aggaggaggggaggagaggg

SEQ ID NO: 10964 - RNA, 20 nt, synthetic construct
  source 1..20: mol_type = other RNA
gtgaggaggaggggaggaga

SEQ ID NO: 10965 - RNA, 20 nt, synthetic construct
  source 1..20: mol_type = other RNA
cgtgaggaggaggggaggag

SEQ ID NO: 10966 - RNA, 20 nt, synthetic construct
  source 1..20: mol_type = other RNA
aaggtcgtgaggaggagggg

SEQ ID NO: 10967 - RNA, 20 nt, synthetic construct
  source 1..20: mol_type = other RNA
agaaaggtcgtgaggaggag

SEQ ID NO: 10968 - RNA, 20 nt, synthetic construct
  source 1..20: mol_type = other RNA
gagaaaggtcgtgaggagga

SEQ ID NO: 10969 - RNA, 20 nt, synthetic construct
  source 1..20: mol_type = other RNA
agagaaaggtcgtgaggagg

SEQ ID NO: 10970 - RNA, 20 nt, synthetic construct
  source 1..20: mol_type = other RNA
gagagagaaaggtcgtgagg

SEQ ID NO: 10971 - RNA, 20 nt, synthetic construct
  source 1..20: mol_type = other RNA
agggagagagaaaggtcgtg

SEQ ID NO: 10972 - RNA, 20 nt, synthetic construct
  source 1..20: mol_type = other RNA
gcaacttgagggagagagaa

SEQ ID NO: 10973 - RNA, 20 nt, synthetic construct
  source 1..20: mol_type = other RNA
ctcaagttgccatctgcacg

SEQ ID NO: 10974 - RNA, 20 nt, synthetic construct
  source 1..20: mol_type = other RNA
tcgtgcagatggcaacttga

SEQ ID NO: 10975 - RNA, 20 nt, synthetic construct
  source 1..20: mol_type = other RNA
ctcgtgcagatggcaacttg

SEQ ID NO: 10976 - RNA, 20 nt, synthetic construct
  source 1..20: mol_type = other RNA
catctgcacgaggtcagagc

SEQ ID NO: 10977 - RNA, 20 nt, synthetic construct
  source 1..20: mol_type = other RNA
ctgcacgaggtcagagctgg

SEQ ID NO: 10978 - RNA, 20 nt, synthetic construct
  source 1..20: mol_type = other RNA
cagctctgacctcgtgcaga

SEQ ID NO: 10979 - RNA, 20 nt, synthetic construct
  source 1..20: mol_type = other RNA
ggaggatttcctgagtgaag

SEQ ID NO: 10980 - RNA, 20 nt, synthetic construct
  source 1..20: mol_type = other RNA
gagtgaagcggtctgcatga

SEQ ID NO: 10981 - RNA, 20 nt, synthetic construct
  source 1..20: mol_type = other RNA
tcatgcagaccgcttcactc

SEQ ID NO: 10982 - RNA, 20 nt, synthetic construct
  source 1..20: mol_type = other RNA
ttgaccatcccaacgtcatg

SEQ ID NO: 10983 - RNA, 20 nt, synthetic construct
  source 1..20: mol_type = other RNA
cccaacgtcatgaggctcat

SEQ ID NO: 10984 - RNA, 20 nt, synthetic construct
  source 1..20: mol_type = other RNA
tgagcctcatgacgttggga

SEQ ID NO: 10985 - RNA, 20 nt, synthetic construct
  source 1..20: mol_type = other RNA
ccgatgagcctcatgacgtt

SEQ ID NO: 10986 - RNA, 20 nt, synthetic construct
  source 1..20: mol_type = other RNA
accgatgagcctcatgacgt

SEQ ID NO: 10987 - RNA, 20 nt, synthetic construct
  source 1..20: mol_type = other RNA
atgaggctcatcggtgagag

SEQ ID NO: 10988 - RNA, 20 nt, synthetic construct
  source 1..20: mol_type = other RNA
tgaggctcatcggtgagaga

SEQ ID NO: 10989 - RNA, 20 nt, synthetic construct
  source 1..20: mol_type = other RNA
gaggctcatcggtgagagag

SEQ ID NO: 10990 - RNA, 20 nt, synthetic construct
  source 1..20: mol_type = other RNA
gtgagagaggggcagattca

SEQ ID NO: 10991 - RNA, 20 nt, synthetic construct
  source 1..20: mol_type = other RNA
tgagagaggggcagattcaa

SEQ ID NO: 10992 - RNA, 20 nt, synthetic construct
  source 1..20: mol_type = other RNA
gagagaggggcagattcaag

SEQ ID NO: 10993 - RNA, 20 nt, synthetic construct
  source 1..20: mol_type = other RNA
caaggggtctacaagcccca

SEQ ID NO: 10994 - RNA, 20 nt, synthetic construct
  source 1..20: mol_type = other RNA
aaggggtctacaagccccat

SEQ ID NO: 10995 - RNA, 20 nt, synthetic construct
  source 1..20: mol_type = other RNA
aggggtctacaagccccatg

SEQ ID NO: 10996 - RNA, 20 nt, synthetic construct
  source 1..20: mol_type = other RNA
ggggtctacaagccccatgg

SEQ ID NO: 10997 - RNA, 20 nt, synthetic construct
  source 1..20: mol_type = other RNA
ccccatgggggccatagcag

SEQ ID NO: 10998 - RNA, 20 nt, synthetic construct
  source 1..20: mol_type = other RNA
cccatgggggccatagcaga

SEQ ID NO: 10999 - RNA, 20 nt, synthetic construct
  source 1..20: mol_type = other RNA
cctctgctatggcccccatg

SEQ ID NO: 11000 - RNA, 20 nt, synthetic construct
  source 1..20: mol_type = other RNA
ccctctgctatggcccccat

SEQ ID NO: 11001 - RNA, 20 nt, synthetic construct
  source 1..20: mol_type = other RNA
tccctctgctatggccccca

SEQ ID NO: 11002 - RNA, 20 nt, synthetic construct
  source 1..20: mol_type = other RNA
cagggctcttccctctgcta

SEQ ID NO: 11003 - RNA, 20 nt, synthetic construct
  source 1..20: mol_type = other RNA
agagggaagagccctgcttc

SEQ ID NO: 11004 - RNA, 20 nt, synthetic construct
  source 1..20: mol_type = other RNA
aagagccctgcttctggccc

SEQ ID NO: 11005 - RNA, 20 nt, synthetic construct
  source 1..20: mol_type = other RNA
agagccctgcttctggccct

SEQ ID NO: 11006 - RNA, 20 nt, synthetic construct
  source 1..20: mol_type = other RNA
tcttcccagggccagaagca

SEQ ID NO: 11007 - RNA, 20 nt, synthetic construct
  source 1..20: mol_type = other RNA
atcttcccagggccagaagc

SEQ ID NO: 11008 - RNA, 20 nt, synthetic construct
  source 1..20: mol_type = other RNA
cctgggaagatcaaacttcc

SEQ ID NO: 11009 - RNA, 20 nt, synthetic construct
  source 1..20: mol_type = other RNA
ctggaagtttgatcttccca

SEQ ID NO: 11010 - RNA, 20 nt, synthetic construct
  source 1..20: mol_type = other RNA
cctggaagtttgatcttccc

SEQ ID NO: 11011 - RNA, 20 nt, synthetic construct
  source 1..20: mol_type = other RNA
ggagcggggagcaggaagcc

SEQ ID NO: 11012 - RNA, 20 nt, synthetic construct
  source 1..20: mol_type = other RNA
ttcctgctccccgctccttc

SEQ ID NO: 11013 - RNA, 20 nt, synthetic construct
  source 1..20: mol_type = other RNA
tcctgctccccgctccttca

SEQ ID NO: 11014 - RNA, 20 nt, synthetic construct
  source 1..20: mol_type = other RNA
ctggccaccatattgtttgg

SEQ ID NO: 11015 - RNA, 20 nt, synthetic construct
  source 1..20: mol_type = other RNA
tctggccaccatattgtttg

SEQ ID NO: 11016 - RNA, 20 nt, synthetic construct
  source 1..20: mol_type = other RNA
atctggccaccatattgttt

SEQ ID NO: 11017 - RNA, 20 nt, synthetic construct
  source 1..20: mol_type = other RNA
aatctggccaccatattgtt

SEQ ID NO: 11018 - RNA, 20 nt, synthetic construct
  source 1..20: mol_type = other RNA
aatatggtggccagattgga

SEQ ID NO: 11019 - RNA, 20 nt, synthetic construct
  source 1..20: mol_type = other RNA
atatggtggccagattggat

SEQ ID NO: 11020 - RNA, 20 nt, synthetic construct
  source 1..20: mol_type = other RNA
agattggatgggtagtgaga

SEQ ID NO: 11021 - RNA, 20 nt, synthetic construct
  source 1..20: mol_type = other RNA
ttctcactacccatccaatc

SEQ ID NO: 11022 - RNA, 20 nt, synthetic construct
  source 1..20: mol_type = other RNA
ggatgggtagtgagaaggag

SEQ ID NO: 11023 - RNA, 20 nt, synthetic construct
  source 1..20: mol_type = other RNA
gggtagtgagaaggagaggc

SEQ ID NO: 11024 - RNA, 20 nt, synthetic construct
  source 1..20: mol_type = other RNA
tagtgagaaggagaggctgg

SEQ ID NO: 11025 - RNA, 20 nt, synthetic construct
  source 1..20: mol_type = other RNA
gagaaggagaggctggaggc

SEQ ID NO: 11026 - RNA, 20 nt, synthetic construct
  source 1..20: mol_type = other RNA
aggagaggctggaggctggc

SEQ ID NO: 11027 - RNA, 20 nt, synthetic construct
  source 1..20: mol_type = other RNA
agaggctggaggctggctgg

SEQ ID NO: 11028 - RNA, 20 nt, synthetic construct
  source 1..20: mol_type = other RNA
gaggctggaggctggctggt

SEQ ID NO: 11029 - RNA, 20 nt, synthetic construct
  source 1..20: mol_type = other RNA
aggctggaggctggctggtg

SEQ ID NO: 11030 - RNA, 20 nt, synthetic construct
  source 1..20: mol_type = other RNA
ggctggaggctggctggtgg

SEQ ID NO: 11031 - RNA, 20 nt, synthetic construct
  source 1..20: mol_type = other RNA
gctggaggctggctggtggg

SEQ ID NO: 11032 - RNA, 20 nt, synthetic construct
  source 1..20: mol_type = other RNA
aggctggctggtggggggct

SEQ ID NO: 11033 - RNA, 20 nt, synthetic construct
  source 1..20: mol_type = other RNA
ggcttccccttctgcccagc

SEQ ID NO: 11034 - RNA, 20 nt, synthetic construct
  source 1..20: mol_type = other RNA
ttctgcccagcaggagtgac

SEQ ID NO: 11035 - RNA, 20 nt, synthetic construct
  source 1..20: mol_type = other RNA
tctgcccagcaggagtgaca

SEQ ID NO: 11036 - RNA, 20 nt, synthetic construct
  source 1..20: mol_type = other RNA
gtcactcctgctgggcagaa

SEQ ID NO: 11037 - RNA, 20 nt, synthetic construct
  source 1..20: mol_type = other RNA
tgtcactcctgctgggcaga

SEQ ID NO: 11038 - RNA, 20 nt, synthetic construct
  source 1..20: mol_type = other RNA
gcaggagtgacagggctacc

SEQ ID NO: 11039 - RNA, 20 nt, synthetic construct
  source 1..20: mol_type = other RNA
gtagccctgtcactcctgct

SEQ ID NO: 11040 - RNA, 20 nt, synthetic construct
  source 1..20: mol_type = other RNA
aggagtgacagggctacctg

SEQ ID NO: 11041 - RNA, 20 nt, synthetic construct
  source 1..20: mol_type = other RNA
ggagtgacagggctacctgg

SEQ ID NO: 11042 - RNA, 20 nt, synthetic construct
  source 1..20: mol_type = other RNA
gagtgacagggctacctggg

SEQ ID NO: 11043 - RNA, 20 nt, synthetic construct
  source 1..20: mol_type = other RNA
cagggctacctggggggctc

SEQ ID NO: 11044 - RNA, 20 nt, synthetic construct
  source 1..20: mol_type = other RNA
aacagacacctgagcccccc

SEQ ID NO: 11045 - RNA, 20 nt, synthetic construct
  source 1..20: mol_type = other RNA
gggctcaggtgtctgtttcc

SEQ ID NO: 11046 - RNA, 20 nt, synthetic construct
  source 1..20: mol_type = other RNA
ggctcaggtgtctgtttcca

SEQ ID NO: 11047 - RNA, 20 nt, synthetic construct
  source 1..20: mol_type = other RNA
agctctctcgttcagaaccc

SEQ ID NO: 11048 - RNA, 20 nt, synthetic construct
  source 1..20: mol_type = other RNA
agagagcttcccagcacctg

SEQ ID NO: 11049 - RNA, 20 nt, synthetic construct
  source 1..20: mol_type = other RNA
gtaagatgaccacaggtgct

SEQ ID NO: 11050 - RNA, 20 nt, synthetic construct
  source 1..20: mol_type = other RNA
ggtaagatgaccacaggtgc

SEQ ID NO: 11051 - RNA, 20 nt, synthetic construct
  source 1..20: mol_type = other RNA
atgaaaggtaagatgaccac

SEQ ID NO: 11052 - RNA, 20 nt, synthetic construct
  source 1..20: mol_type = other RNA
atcttacctttcatgaaaca

SEQ ID NO: 11053 - RNA, 20 nt, synthetic construct
  source 1..20: mol_type = other RNA
aggtctccatgtttcatgaa

SEQ ID NO: 11054 - RNA, 20 nt, synthetic construct
  source 1..20: mol_type = other RNA
aatagaggaggaagctgtgt

SEQ ID NO: 11055 - RNA, 20 nt, synthetic construct
  source 1..20: mol_type = other RNA
ttcctcctctattcccggct

SEQ ID NO: 11056 - RNA, 20 nt, synthetic construct
  source 1..20: mol_type = other RNA
tcctcctctattcccggctc

SEQ ID NO: 11057 - RNA, 20 nt, synthetic construct
  source 1..20: mol_type = other RNA
cctcctctattcccggctcg

SEQ ID NO: 11058 - RNA, 20 nt, synthetic construct
  source 1..20: mol_type = other RNA
ccccgagccgggaatagagg

SEQ ID NO: 11059 - RNA, 20 nt, synthetic construct
  source 1..20: mol_type = other RNA
ggtccccgagccgggaatag

SEQ ID NO: 11060 - RNA, 20 nt, synthetic construct
  source 1..20: mol_type = other RNA
ccggctcggggaccagccag

SEQ ID NO: 11061 - RNA, 20 nt, synthetic construct
  source 1..20: mol_type = other RNA
cactggctggtccccgagcc

SEQ ID NO: 11062 - RNA, 20 nt, synthetic construct
  source 1..20: mol_type = other RNA
ccactggctggtccccgagc

SEQ ID NO: 11063 - RNA, 20 nt, synthetic construct
  source 1..20: mol_type = other RNA
cggggaccagccagtggtaa

SEQ ID NO: 11064 - RNA, 20 nt, synthetic construct
  source 1..20: mol_type = other RNA
ggggaccagccagtggtaag

SEQ ID NO: 11065 - RNA, 20 nt, synthetic construct
  source 1..20: mol_type = other RNA
aaacgccccttaccactggc

SEQ ID NO: 11066 - RNA, 20 nt, synthetic construct
  source 1..20: mol_type = other RNA
gattaaacgccccttaccac

SEQ ID NO: 11067 - RNA, 20 nt, synthetic construct
  source 1..20: mol_type = other RNA
atattaactgagcatctatc

SEQ ID NO: 11068 - RNA, 20 nt, synthetic construct
  source 1..20: mol_type = other RNA
acccagtgctgctcagaccc

SEQ ID NO: 11069 - RNA, 20 nt, synthetic construct
  source 1..20: mol_type = other RNA
cccagtgctgctcagaccct

SEQ ID NO: 11070 - RNA, 20 nt, synthetic construct
  source 1..20: mol_type = other RNA
cccagggtctgagcagcact

SEQ ID NO: 11071 - RNA, 20 nt, synthetic construct
  source 1..20: mol_type = other RNA
tcccagggtctgagcagcac

SEQ ID NO: 11072 - RNA, 20 nt, synthetic construct
  source 1..20: mol_type = other RNA
ctcagaccctgggaagacca

SEQ ID NO: 11073 - RNA, 20 nt, synthetic construct
  source 1..20: mol_type = other RNA
ctgggaagaccacggtgacc

SEQ ID NO: 11074 - RNA, 20 nt, synthetic construct
  source 1..20: mol_type = other RNA
tggtcaccgtggtcttccca

SEQ ID NO: 11075 - RNA, 20 nt, synthetic construct
  source 1..20: mol_type = other RNA
ctggtcaccgtggtcttccc

SEQ ID NO: 11076 - RNA, 20 nt, synthetic construct
  source 1..20: mol_type = other RNA
gagcaagctcctggtcaccg

SEQ ID NO: 11077 - RNA, 20 nt, synthetic construct
  source 1..20: mol_type = other RNA
tgaccaggagcttgctctcc

SEQ ID NO: 11078 - RNA, 20 nt, synthetic construct
  source 1..20: mol_type = other RNA
gctccaggagagcaagctcc

SEQ ID NO: 11079 - RNA, 20 nt, synthetic construct
  source 1..20: mol_type = other RNA
agggccatgggaaaccactg

SEQ ID NO: 11080 - RNA, 20 nt, synthetic construct
  source 1..20: mol_type = other RNA
gggccatgggaaaccactgc

SEQ ID NO: 11081 - RNA, 20 nt, synthetic construct
  source 1..20: mol_type = other RNA
ctgcccgcagtggtttccca

SEQ ID NO: 11082 - RNA, 20 nt, synthetic construct
  source 1..20: mol_type = other RNA
aaaccactgcgggcagagct

SEQ ID NO: 11083 - RNA, 20 nt, synthetic construct
  source 1..20: mol_type = other RNA
aagcctagctctgcccgcag

SEQ ID NO: 11084 - RNA, 20 nt, synthetic construct
  source 1..20: mol_type = other RNA
gcagagctaggcttgcacag

SEQ ID NO: 11085 - RNA, 20 nt, synthetic construct
  source 1..20: mol_type = other RNA
cagagctaggcttgcacaga

SEQ ID NO: 11086 - RNA, 20 nt, synthetic construct
  source 1..20: mol_type = other RNA
gctaggcttgcacagaggga

SEQ ID NO: 11087 - RNA, 20 nt, synthetic construct
  source 1..20: mol_type = other RNA
aggcttgcacagagggatgg

SEQ ID NO: 11088 - RNA, 20 nt, synthetic construct
  source 1..20: mol_type = other RNA
ggcttgcacagagggatgga

SEQ ID NO: 11089 - RNA, 20 nt, synthetic construct
  source 1..20: mol_type = other RNA
ttgcacagagggatggaggg

SEQ ID NO: 11090 - RNA, 20 nt, synthetic construct
  source 1..20: mol_type = other RNA
cacagagggatggagggagg

SEQ ID NO: 11091 - RNA, 20 nt, synthetic construct
  source 1..20: mol_type = other RNA
acagagggatggagggagga

SEQ ID NO: 11092 - RNA, 20 nt, synthetic construct
  source 1..20: mol_type = other RNA
agggaggagggatcgcatca

SEQ ID NO: 11093 - RNA, 20 nt, synthetic construct
  source 1..20: mol_type = other RNA
acctctcctcccacctgcct

SEQ ID NO: 11094 - RNA, 20 nt, synthetic construct
  source 1..20: mol_type = other RNA
gccaaggcaggtgggaggag

SEQ ID NO: 11095 - RNA, 20 nt, synthetic construct
  source 1..20: mol_type = other RNA
ggggagccaaggcaggtggg

SEQ ID NO: 11096 - RNA, 20 nt, synthetic construct
  source 1..20: mol_type = other RNA
actggggagccaaggcaggt

SEQ ID NO: 11097 - RNA, 20 nt, synthetic construct
  source 1..20: mol_type = other RNA
tactggggagccaaggcagg

SEQ ID NO: 11098 - RNA, 20 nt, synthetic construct
  source 1..20: mol_type = other RNA
aggtactggggagccaaggc

SEQ ID NO: 11099 - RNA, 20 nt, synthetic construct
  source 1..20: mol_type = other RNA
gggcaggtactggggagcca

SEQ ID NO: 11100 - RNA, 20 nt, synthetic construct
  source 1..20: mol_type = other RNA
atctgagtgggcaggtactg

SEQ ID NO: 11101 - RNA, 20 nt, synthetic construct
  source 1..20: mol_type = other RNA
catctgagtgggcaggtact

SEQ ID NO: 11102 - RNA, 20 nt, synthetic construct
  source 1..20: mol_type = other RNA
gcatctgagtgggcaggtac

SEQ ID NO: 11103 - RNA, 20 nt, synthetic construct
  source 1..20: mol_type = other RNA
tcactagcatctgagtgggc

SEQ ID NO: 11104 - RNA, 20 nt, synthetic construct
  source 1..20: mol_type = other RNA
tcagatgctagtgaagttca

SEQ ID NO: 11105 - RNA, 20 nt, synthetic construct
  source 1..20: mol_type = other RNA
gaacttcactagcatctgag

SEQ ID NO: 11106 - RNA, 20 nt, synthetic construct
  source 1..20: mol_type = other RNA
ttcatggcagacatcgccag

SEQ ID NO: 11107 - RNA, 20 nt, synthetic construct
  source 1..20: mol_type = other RNA
ggcagacatcgccagtggca

SEQ ID NO: 11108 - RNA, 20 nt, synthetic construct
  source 1..20: mol_type = other RNA
actcagatactccatgccac

SEQ ID NO: 11109 - RNA, 20 nt, synthetic construct
  source 1..20: mol_type = other RNA
gtaccaagagattcatacac

SEQ ID NO: 11110 - RNA, 20 nt, synthetic construct
  source 1..20: mol_type = other RNA
taccaagagattcatacacc

SEQ ID NO: 11111 - RNA, 20 nt, synthetic construct
  source 1..20: mol_type = other RNA
gagattcatacaccgggacc

SEQ ID NO: 11112 - RNA, 20 nt, synthetic construct
  source 1..20: mol_type = other RNA
gtcccggtgtatgaatctct

SEQ ID NO: 11113 - RNA, 20 nt, synthetic construct
  source 1..20: mol_type = other RNA
attcatacaccgggacctgg

SEQ ID NO: 11114 - RNA, 20 nt, synthetic construct
  source 1..20: mol_type = other RNA
tacaccgggacctggcggcc

SEQ ID NO: 11115 - RNA, 20 nt, synthetic construct
  source 1..20: mol_type = other RNA
agttcctggccgccaggtcc

SEQ ID NO: 11116 - RNA, 20 nt, synthetic construct
  source 1..20: mol_type = other RNA
acatgcagttcctggccgcc

SEQ ID NO: 11117 - RNA, 20 nt, synthetic construct
  source 1..20: mol_type = other RNA
aggcactcacatgcagttcc

SEQ ID NO: 11118 - RNA, 20 nt, synthetic construct
  source 1..20: mol_type = other RNA
actgcatgtgagtgcctttc

SEQ ID NO: 11119 - RNA, 20 nt, synthetic construct
  source 1..20: mol_type = other RNA
ctgcatgtgagtgcctttca

SEQ ID NO: 11120 - RNA, 20 nt, synthetic construct
  source 1..20: mol_type = other RNA
ggggggggggggtccctgaa

SEQ ID NO: 11121 - RNA, 20 nt, synthetic construct
  source 1..20: mol_type = other RNA
caggagcagttggggggggg

SEQ ID NO: 11122 - RNA, 20 nt, synthetic construct
  source 1..20: mol_type = other RNA
gcaggagcagttgggggggg

SEQ ID NO: 11123 - RNA, 20 nt, synthetic construct
  source 1..20: mol_type = other RNA
tgcaggagcagttggggggg

SEQ ID NO: 11124 - RNA, 20 nt, synthetic construct
  source 1..20: mol_type = other RNA
gtgcaggagcagttgggggg

SEQ ID NO: 11125 - RNA, 20 nt, synthetic construct
  source 1..20: mol_type = other RNA
agtgcaggagcagttggggg

SEQ ID NO: 11126 - RNA, 20 nt, synthetic construct
  source 1..20: mol_type = other RNA
gagtgcaggagcagttgggg

SEQ ID NO: 11127 - RNA, 20 nt, synthetic construct
  source 1..20: mol_type = other RNA
ggagtgcaggagcagttggg

SEQ ID NO: 11128 - RNA, 20 nt, synthetic construct
  source 1..20: mol_type = other RNA
gggagtgcaggagcagttgg

SEQ ID NO: 11129 - RNA, 20 nt, synthetic construct
  source 1..20: mol_type = other RNA
actgctcctgcactccctga

SEQ ID NO: 11130 - RNA, 20 nt, synthetic construct
  source 1..20: mol_type = other RNA
cagggagtgcaggagcagtt

SEQ ID NO: 11131 - RNA, 20 nt, synthetic construct
  source 1..20: mol_type = other RNA
tcagggagtgcaggagcagt

SEQ ID NO: 11132 - RNA, 20 nt, synthetic construct
  source 1..20: mol_type = other RNA
ggaactccctcagggagtgc

SEQ ID NO: 11133 - RNA, 20 nt, synthetic construct
  source 1..20: mol_type = other RNA
ggagggagggaactccctca

SEQ ID NO: 11134 - RNA, 20 nt, synthetic construct
  source 1..20: mol_type = other RNA
aggagggagggaactccctc

SEQ ID NO: 11135 - RNA, 20 nt, synthetic construct
  source 1..20: mol_type = other RNA
gagttccctccctccttctt

SEQ ID NO: 11136 - RNA, 20 nt, synthetic construct
  source 1..20: mol_type = other RNA
tccctccctccttcttagga

SEQ ID NO: 11137 - RNA, 20 nt, synthetic construct
  source 1..20: mol_type = other RNA
tccatcctaagaaggaggga

SEQ ID NO: 11138 - RNA, 20 nt, synthetic construct
  source 1..20: mol_type = other RNA
ctccttcttaggatggaagc

SEQ ID NO: 11139 - RNA, 20 nt, synthetic construct
  source 1..20: mol_type = other RNA
tccttcttaggatggaagca

SEQ ID NO: 11140 - RNA, 20 nt, synthetic construct
  source 1..20: mol_type = other RNA
tgcttccatcctaagaagga

SEQ ID NO: 11141 - RNA, 20 nt, synthetic construct
  source 1..20: mol_type = other RNA
ctgcttccatcctaagaagg

SEQ ID NO: 11142 - RNA, 20 nt, synthetic construct
  source 1..20: mol_type = other RNA
gccctgcttccatcctaaga

SEQ ID NO: 11143 - RNA, 20 nt, synthetic construct
  source 1..20: mol_type = other RNA
gcagggctagacacccgctg

SEQ ID NO: 11144 - RNA, 20 nt, synthetic construct
  source 1..20: mol_type = other RNA
cagggctagacacccgctga

SEQ ID NO: 11145 - RNA, 20 nt, synthetic construct
  source 1..20: mol_type = other RNA
gctagacacccgctgagggc

SEQ ID NO: 11146 - RNA, 20 nt, synthetic construct
  source 1..20: mol_type = other RNA
ctgagggcaggtcagaactc

SEQ ID NO: 11147 - RNA, 20 nt, synthetic construct
  source 1..20: mol_type = other RNA
agttctgacctgccctcagc

SEQ ID NO: 11148 - RNA, 20 nt, synthetic construct
  source 1..20: mol_type = other RNA
gagttctgacctgccctcag

SEQ ID NO: 11149 - RNA, 20 nt, synthetic construct
  source 1..20: mol_type = other RNA
cacccgcagccaggacagtg

SEQ ID NO: 11150 - RNA, 20 nt, synthetic construct
  source 1..20: mol_type = other RNA
acccgcagccaggacagtga

SEQ ID NO: 11151 - RNA, 20 nt, synthetic construct
  source 1..20: mol_type = other RNA
cactgtcctggctgcgggtg

SEQ ID NO: 11152 - RNA, 20 nt, synthetic construct
  source 1..20: mol_type = other RNA
tcactgtcctggctgcgggt

SEQ ID NO: 11153 - RNA, 20 nt, synthetic construct
  source 1..20: mol_type = other RNA
ctcactgtcctggctgcggg

SEQ ID NO: 11154 - RNA, 20 nt, synthetic construct
  source 1..20: mol_type = other RNA
gcagccaggacagtgagggg

SEQ ID NO: 11155 - RNA, 20 nt, synthetic construct
  source 1..20: mol_type = other RNA
cccctcactgtcctggctgc

SEQ ID NO: 11156 - RNA, 20 nt, synthetic construct
  source 1..20: mol_type = other RNA
tcccctcactgtcctggctg

SEQ ID NO: 11157 - RNA, 20 nt, synthetic construct
  source 1..20: mol_type = other RNA
acctcctcccctcactgtcc

SEQ ID NO: 11158 - RNA, 20 nt, synthetic construct
  source 1..20: mol_type = other RNA
tgcagatgtgtctgagagcc

SEQ ID NO: 11159 - RNA, 20 nt, synthetic construct
  source 1..20: mol_type = other RNA
gcagatgtgtctgagagcca

SEQ ID NO: 11160 - RNA, 20 nt, synthetic construct
  source 1..20: mol_type = other RNA
atgtgtctgagagccagggc

SEQ ID NO: 11161 - RNA, 20 nt, synthetic construct
  source 1..20: mol_type = other RNA
gagagccagggcaggcttcc

SEQ ID NO: 11162 - RNA, 20 nt, synthetic construct
  source 1..20: mol_type = other RNA
agccagggcaggcttcctgg

SEQ ID NO: 11163 - RNA, 20 nt, synthetic construct
  source 1..20: mol_type = other RNA
cagggcaggcttcctggtgg

SEQ ID NO: 11164 - RNA, 20 nt, synthetic construct
  source 1..20: mol_type = other RNA
ctccaccaggaagcctgccc

SEQ ID NO: 11165 - RNA, 20 nt, synthetic construct
  source 1..20: mol_type = other RNA
gggcatcagtcacctccacc

SEQ ID NO: 11166 - RNA, 20 nt, synthetic construct
  source 1..20: mol_type = other RNA
tggggaaaggaacagggtca

SEQ ID NO: 11167 - RNA, 20 nt, synthetic construct
  source 1..20: mol_type = other RNA
ttggggaaaggaacagggtc

SEQ ID NO: 11168 - RNA, 20 nt, synthetic construct
  source 1..20: mol_type = other RNA
ttcctttccccaatccaaac

SEQ ID NO: 11169 - RNA, 20 nt, synthetic construct
  source 1..20: mol_type = other RNA
tttggattggggaaaggaac

SEQ ID NO: 11170 - RNA, 20 nt, synthetic construct
  source 1..20: mol_type = other RNA
agcctgtttggattggggaa

SEQ ID NO: 11171 - RNA, 20 nt, synthetic construct
  source 1..20: mol_type = other RNA
cattcagcctgtttggattg

SEQ ID NO: 11172 - RNA, 20 nt, synthetic construct
  source 1..20: mol_type = other RNA
tcattcagcctgtttggatt

SEQ ID NO: 11173 - RNA, 20 nt, synthetic construct
  source 1..20: mol_type = other RNA
ctcattcagcctgtttggat

SEQ ID NO: 11174 - RNA, 20 nt, synthetic construct
  source 1..20: mol_type = other RNA
atgttctcattcagcctgtt

SEQ ID NO: 11175 - RNA, 20 nt, synthetic construct
  source 1..20: mol_type = other RNA
tgagaacatgtccgtgtgtg

SEQ ID NO: 11176 - RNA, 20 nt, synthetic construct
  source 1..20: mol_type = other RNA
gaacatgtccgtgtgtgtgg

SEQ ID NO: 11177 - RNA, 20 nt, synthetic construct
  source 1..20: mol_type = other RNA
tccgtgtgtgtggcggactt

SEQ ID NO: 11178 - RNA, 20 nt, synthetic construct
  source 1..20: mol_type = other RNA
ccgtgtgtgtggcggacttc

SEQ ID NO: 11179 - RNA, 20 nt, synthetic construct
  source 1..20: mol_type = other RNA
cccgaagtccgccacacaca

SEQ ID NO: 11180 - RNA, 20 nt, synthetic construct
  source 1..20: mol_type = other RNA
ctctccaagaagatctacaa

SEQ ID NO: 11181 - RNA, 20 nt, synthetic construct
  source 1..20: mol_type = other RNA
tctccaagaagatctacaat

SEQ ID NO: 11182 - RNA, 20 nt, synthetic construct
  source 1..20: mol_type = other RNA
ctccaagaagatctacaatg

SEQ ID NO: 11183 - RNA, 20 nt, synthetic construct
  source 1..20: mol_type = other RNA
gtccccattgtagatcttct

SEQ ID NO: 11184 - RNA, 20 nt, synthetic construct
  source 1..20: mol_type = other RNA
caatggggactactaccgcc

SEQ ID NO: 11185 - RNA, 20 nt, synthetic construct
  source 1..20: mol_type = other RNA
aatggggactactaccgcca

SEQ ID NO: 11186 - RNA, 20 nt, synthetic construct
  source 1..20: mol_type = other RNA
tcttggcgatacgtccctgg

SEQ ID NO: 11187 - RNA, 20 nt, synthetic construct
  source 1..20: mol_type = other RNA
gcatcttggcgatacgtccc

SEQ ID NO: 11188 - RNA, 20 nt, synthetic construct
  source 1..20: mol_type = other RNA
tcgccaagatgccagtcaag

SEQ ID NO: 11189 - RNA, 20 nt, synthetic construct
  source 1..20: mol_type = other RNA
aatccacttgactggcatct

SEQ ID NO: 11190 - RNA, 20 nt, synthetic construct
  source 1..20: mol_type = other RNA
tcaatggcaatccacttgac

SEQ ID NO: 11191 - RNA, 20 nt, synthetic construct
  source 1..20: mol_type = other RNA
acggtcagctagactctcaa

SEQ ID NO: 11192 - RNA, 20 nt, synthetic construct
  source 1..20: mol_type = other RNA
cgctcttgctggtgtagaca

SEQ ID NO: 11193 - RNA, 20 nt, synthetic construct
  source 1..20: mol_type = other RNA
ctacaccagcaagagcgatg

SEQ ID NO: 11194 - RNA, 20 nt, synthetic construct
  source 1..20: mol_type = other RNA
accagcaagagcgatgtggt

SEQ ID NO: 11195 - RNA, 20 nt, synthetic construct
  source 1..20: mol_type = other RNA
acctaccacatcgctcttgc

SEQ ID NO: 11196 - RNA, 20 nt, synthetic construct
  source 1..20: mol_type = other RNA
aggtgcactcccgccaagag

SEQ ID NO: 11197 - RNA, 20 nt, synthetic construct
  source 1..20: mol_type = other RNA
ggtgcactcccgccaagagt

SEQ ID NO: 11198 - RNA, 20 nt, synthetic construct
  source 1..20: mol_type = other RNA
gtgcactcccgccaagagtg

SEQ ID NO: 11199 - RNA, 20 nt, synthetic construct
  source 1..20: mol_type = other RNA
ccgccaagagtggggaacca

SEQ ID NO: 11200 - RNA, 20 nt, synthetic construct
  source 1..20: mol_type = other RNA
cgccaagagtggggaaccat

SEQ ID NO: 11201 - RNA, 20 nt, synthetic construct
  source 1..20: mol_type = other RNA
caagagtggggaaccatggg

SEQ ID NO: 11202 - RNA, 20 nt, synthetic construct
  source 1..20: mol_type = other RNA
aagagtggggaaccatggga

SEQ ID NO: 11203 - RNA, 20 nt, synthetic construct
  source 1..20: mol_type = other RNA
ctcccatggttccccactct

SEQ ID NO: 11204 - RNA, 20 nt, synthetic construct
  source 1..20: mol_type = other RNA
tggggaaccatgggagggca

SEQ ID NO: 11205 - RNA, 20 nt, synthetic construct
  source 1..20: mol_type = other RNA
ggtcaggccatgccctccca

SEQ ID NO: 11206 - RNA, 20 nt, synthetic construct
  source 1..20: mol_type = other RNA
tgaccatcacacactatgcc

SEQ ID NO: 11207 - RNA, 20 nt, synthetic construct
  source 1..20: mol_type = other RNA
gaccatcacacactatgcct

SEQ ID NO: 11208 - RNA, 20 nt, synthetic construct
  source 1..20: mol_type = other RNA
aggcatagtgtgtgatggtc

SEQ ID NO: 11209 - RNA, 20 nt, synthetic construct
  source 1..20: mol_type = other RNA
catcacacactatgcctggg

SEQ ID NO: 11210 - RNA, 20 nt, synthetic construct
  source 1..20: mol_type = other RNA
cacccaggcatagtgtgtga

SEQ ID NO: 11211 - RNA, 20 nt, synthetic construct
  source 1..20: mol_type = other RNA
acactatgcctgggtggctg

SEQ ID NO: 11212 - RNA, 20 nt, synthetic construct
  source 1..20: mol_type = other RNA
cctgggtggctgtggatgca

SEQ ID NO: 11213 - RNA, 20 nt, synthetic construct
  source 1..20: mol_type = other RNA
ctgggtggctgtggatgcaa

SEQ ID NO: 11214 - RNA, 20 nt, synthetic construct
  source 1..20: mol_type = other RNA
ccttgcatccacagccaccc

SEQ ID NO: 11215 - RNA, 20 nt, synthetic construct
  source 1..20: mol_type = other RNA
gctgtggatgcaagggtcac

SEQ ID NO: 11216 - RNA, 20 nt, synthetic construct
  source 1..20: mol_type = other RNA
ctgtggatgcaagggtcaca

SEQ ID NO: 11217 - RNA, 20 nt, synthetic construct
  source 1..20: mol_type = other RNA
gcaagggtcacagggacatg

SEQ ID NO: 11218 - RNA, 20 nt, synthetic construct
  source 1..20: mol_type = other RNA
caagggtcacagggacatgt

SEQ ID NO: 11219 - RNA, 20 nt, synthetic construct
  source 1..20: mol_type = other RNA
acatgtgggcttccctttgc

SEQ ID NO: 11220 - RNA, 20 nt, synthetic construct
  source 1..20: mol_type = other RNA
catgtgggcttccctttgca

SEQ ID NO: 11221 - RNA, 20 nt, synthetic construct
  source 1..20: mol_type = other RNA
atgtgggcttccctttgcag

SEQ ID NO: 11222 - RNA, 20 nt, synthetic construct
  source 1..20: mol_type = other RNA
catgttcacaaccatcctct

SEQ ID NO: 11223 - RNA, 20 nt, synthetic construct
  source 1..20: mol_type = other RNA
acatgttcacaaccatcctc

SEQ ID NO: 11224 - RNA, 20 nt, synthetic construct
  source 1..20: mol_type = other RNA
tgaacatgtgtacataagtg

SEQ ID NO: 11225 - RNA, 20 nt, synthetic construct
  source 1..20: mol_type = other RNA
gaacatgtgtacataagtgt

SEQ ID NO: 11226 - RNA, 20 nt, synthetic construct
  source 1..20: mol_type = other RNA
tgtgggtgtacccatgaacc

SEQ ID NO: 11227 - RNA, 20 nt, synthetic construct
  source 1..20: mol_type = other RNA
gtgggtgtacccatgaacct

SEQ ID NO: 11228 - RNA, 20 nt, synthetic construct
  source 1..20: mol_type = other RNA
gtacccatgaacctgggtat

SEQ ID NO: 11229 - RNA, 20 nt, synthetic construct
  source 1..20: mol_type = other RNA
catgaacctgggtattggtg

SEQ ID NO: 11230 - RNA, 20 nt, synthetic construct
  source 1..20: mol_type = other RNA
atgaacctgggtattggtgc

SEQ ID NO: 11231 - RNA, 20 nt, synthetic construct
  source 1..20: mol_type = other RNA
gcaccaatacccaggttcat

SEQ ID NO: 11232 - RNA, 20 nt, synthetic construct
  source 1..20: mol_type = other RNA
cgcaccaatacccaggttca

SEQ ID NO: 11233 - RNA, 20 nt, synthetic construct
  source 1..20: mol_type = other RNA
aatcacccgcaccaataccc

SEQ ID NO: 11234 - RNA, 20 nt, synthetic construct
  source 1..20: mol_type = other RNA
tggtgcgggtgattctgtgc

SEQ ID NO: 11235 - RNA, 20 nt, synthetic construct
  source 1..20: mol_type = other RNA
attccctctgcccctcacag

SEQ ID NO: 11236 - RNA, 20 nt, synthetic construct
  source 1..20: mol_type = other RNA
ggaccactgtgaggggcaga

SEQ ID NO: 11237 - RNA, 20 nt, synthetic construct
  source 1..20: mol_type = other RNA
aggaccactgtgaggggcag

SEQ ID NO: 11238 - RNA, 20 nt, synthetic construct
  source 1..20: mol_type = other RNA
cccctcacagtggtccttcg

SEQ ID NO: 11239 - RNA, 20 nt, synthetic construct
  source 1..20: mol_type = other RNA
ccccgaaggaccactgtgag

SEQ ID NO: 11240 - RNA, 20 nt, synthetic construct
  source 1..20: mol_type = other RNA
accccgaaggaccactgtga

SEQ ID NO: 11241 - RNA, 20 nt, synthetic construct
  source 1..20: mol_type = other RNA
caccccgaaggaccactgtg

SEQ ID NO: 11242 - RNA, 20 nt, synthetic construct
  source 1..20: mol_type = other RNA
ggtccttcggggtgacaatg

SEQ ID NO: 11243 - RNA, 20 nt, synthetic construct
  source 1..20: mol_type = other RNA
gtccttcggggtgacaatgt

SEQ ID NO: 11244 - RNA, 20 nt, synthetic construct
  source 1..20: mol_type = other RNA
ctcccacattgtcaccccga

SEQ ID NO: 11245 - RNA, 20 nt, synthetic construct
  source 1..20: mol_type = other RNA
atgtgggagattgccacaag

SEQ ID NO: 11246 - RNA, 20 nt, synthetic construct
  source 1..20: mol_type = other RNA
aagaggccaaaccccatatc

SEQ ID NO: 11247 - RNA, 20 nt, synthetic construct
  source 1..20: mol_type = other RNA
agaggccaaaccccatatcc

SEQ ID NO: 11248 - RNA, 20 nt, synthetic construct
  source 1..20: mol_type = other RNA
ccaaaccccatatccgggcg

SEQ ID NO: 11249 - RNA, 20 nt, synthetic construct
  source 1..20: mol_type = other RNA
ccacgcccggatatggggtt

SEQ ID NO: 11250 - RNA, 20 nt, synthetic construct
  source 1..20: mol_type = other RNA
gttctccacgcccggatatg

SEQ ID NO: 11251 - RNA, 20 nt, synthetic construct
  source 1..20: mol_type = other RNA
tgttctccacgcccggatat

SEQ ID NO: 11252 - RNA, 20 nt, synthetic construct
  source 1..20: mol_type = other RNA
ctgttctccacgcccggata

SEQ ID NO: 11253 - RNA, 20 nt, synthetic construct
  source 1..20: mol_type = other RNA
atctcgctgttctccacgcc

SEQ ID NO: 11254 - RNA, 20 nt, synthetic construct
  source 1..20: mol_type = other RNA
gatttatgactatctgcgcc

SEQ ID NO: 11255 - RNA, 20 nt, synthetic construct
  source 1..20: mol_type = other RNA
atttatgactatctgcgcca

SEQ ID NO: 11256 - RNA, 20 nt, synthetic construct
  source 1..20: mol_type = other RNA
gctgcttcaggcgatttccc

SEQ ID NO: 11257 - RNA, 20 nt, synthetic construct
  source 1..20: mol_type = other RNA
aaatcgcctgaagcagcctg

SEQ ID NO: 11258 - RNA, 20 nt, synthetic construct
  source 1..20: mol_type = other RNA
gaagcagcctgcggactgtc

SEQ ID NO: 11259 - RNA, 20 nt, synthetic construct
  source 1..20: mol_type = other RNA
gacagtccgcaggctgcttc

SEQ ID NO: 11260 - RNA, 20 nt, synthetic construct
  source 1..20: mol_type = other RNA
cagcctgcggactgtctgga

SEQ ID NO: 11261 - RNA, 20 nt, synthetic construct
  source 1..20: mol_type = other RNA
agtccatccagacagtccgc

SEQ ID NO: 11262 - RNA, 20 nt, synthetic construct
  source 1..20: mol_type = other RNA
gactgtctggatggactgtg

SEQ ID NO: 11263 - RNA, 20 nt, synthetic construct
  source 1..20: mol_type = other RNA
gatggactgtgaggaccctt

SEQ ID NO: 11264 - RNA, 20 nt, synthetic construct
  source 1..20: mol_type = other RNA
ctgggttgggggagacctaa

SEQ ID NO: 11265 - RNA, 20 nt, synthetic construct
  source 1..20: mol_type = other RNA
tctgggttgggggagaccta

SEQ ID NO: 11266 - RNA, 20 nt, synthetic construct
  source 1..20: mol_type = other RNA
tggaatgaattctgggttgg

SEQ ID NO: 11267 - RNA, 20 nt, synthetic construct
  source 1..20: mol_type = other RNA
ttggaatgaattctgggttg

SEQ ID NO: 11268 - RNA, 20 nt, synthetic construct
  source 1..20: mol_type = other RNA
tttggaatgaattctgggtt

SEQ ID NO: 11269 - RNA, 20 nt, synthetic construct
  source 1..20: mol_type = other RNA
gtttggaatgaattctgggt

SEQ ID NO: 11270 - RNA, 20 nt, synthetic construct
  source 1..20: mol_type = other RNA
aggggtttggaatgaattct

SEQ ID NO: 11271 - RNA, 20 nt, synthetic construct
  source 1..20: mol_type = other RNA
caggggtttggaatgaattc

SEQ ID NO: 11272 - RNA, 20 nt, synthetic construct
  source 1..20: mol_type = other RNA
aacccctgactacccccaga

SEQ ID NO: 11273 - RNA, 20 nt, synthetic construct
  source 1..20: mol_type = other RNA
tctgggggtagtcaggggtt

SEQ ID NO: 11274 - RNA, 20 nt, synthetic construct
  source 1..20: mol_type = other RNA
ggccatctgggggtagtcag

SEQ ID NO: 11275 - RNA, 20 nt, synthetic construct
  source 1..20: mol_type = other RNA
gggccatctgggggtagtca

SEQ ID NO: 11276 - RNA, 20 nt, synthetic construct
  source 1..20: mol_type = other RNA
agggccatctgggggtagtc

SEQ ID NO: 11277 - RNA, 20 nt, synthetic construct
  source 1..20: mol_type = other RNA
tacccccagatggccctcac

SEQ ID NO: 11278 - RNA, 20 nt, synthetic construct
  source 1..20: mol_type = other RNA
cagatggccctcacaggtcc

SEQ ID NO: 11279 - RNA, 20 nt, synthetic construct
  source 1..20: mol_type = other RNA
gacctgtgagggccatctgg

SEQ ID NO: 11280 - RNA, 20 nt, synthetic construct
  source 1..20: mol_type = other RNA
ggacctgtgagggccatctg

SEQ ID NO: 11281 - RNA, 20 nt, synthetic construct
  source 1..20: mol_type = other RNA
tggacctgtgagggccatct

SEQ ID NO: 11282 - RNA, 20 nt, synthetic construct
  source 1..20: mol_type = other RNA
ctggacctgtgagggccatc

SEQ ID NO: 11283 - RNA, 20 nt, synthetic construct
  source 1..20: mol_type = other RNA
agagagtcctggacctgtga

SEQ ID NO: 11284 - RNA, 20 nt, synthetic construct
  source 1..20: mol_type = other RNA
tagagagtcctggacctgtg

SEQ ID NO: 11285 - RNA, 20 nt, synthetic construct
  source 1..20: mol_type = other RNA
gtctgggttatagagagtcc

SEQ ID NO: 11286 - RNA, 20 nt, synthetic construct
  source 1..20: mol_type = other RNA
cattctcagggattctgtct

SEQ ID NO: 11287 - RNA, 20 nt, synthetic construct
  source 1..20: mol_type = other RNA
gcattctcagggattctgtc

SEQ ID NO: 11288 - RNA, 20 nt, synthetic construct
  source 1..20: mol_type = other RNA
gggcattttagagggttata

SEQ ID NO: 11289 - RNA, 20 nt, synthetic construct
  source 1..20: mol_type = other RNA
ggggcattttagagggttat

SEQ ID NO: 11290 - RNA, 20 nt, synthetic construct
  source 1..20: mol_type = other RNA
gggactgggggcattttaga

SEQ ID NO: 11291 - RNA, 20 nt, synthetic construct
  source 1..20: mol_type = other RNA
ggggactgggggcattttag

SEQ ID NO: 11292 - RNA, 20 nt, synthetic construct
  source 1..20: mol_type = other RNA
taggacactcaggggactgg

SEQ ID NO: 11293 - RNA, 20 nt, synthetic construct
  source 1..20: mol_type = other RNA
ttaggacactcaggggactg

SEQ ID NO: 11294 - RNA, 20 nt, synthetic construct
  source 1..20: mol_type = other RNA
tttaggacactcaggggact

SEQ ID NO: 11295 - RNA, 20 nt, synthetic construct
  source 1..20: mol_type = other RNA
ttttaggacactcaggggac

SEQ ID NO: 11296 - RNA, 20 nt, synthetic construct
  source 1..20: mol_type = other RNA
gagtgtcctaaaatgtcccc

SEQ ID NO: 11297 - RNA, 20 nt, synthetic construct
  source 1..20: mol_type = other RNA
gggacattttaggacactca

SEQ ID NO: 11298 - RNA, 20 nt, synthetic construct
  source 1..20: mol_type = other RNA
ggggacattttaggacactc

SEQ ID NO: 11299 - RNA, 20 nt, synthetic construct
  source 1..20: mol_type = other RNA
tggaagcctggggacatttt

SEQ ID NO: 11300 - RNA, 20 nt, synthetic construct
  source 1..20: mol_type = other RNA
gggtgcattctggaagcctg

SEQ ID NO: 11301 - RNA, 20 nt, synthetic construct
  source 1..20: mol_type = other RNA
ggggtgcattctggaagcct

SEQ ID NO: 11302 - RNA, 20 nt, synthetic construct
  source 1..20: mol_type = other RNA
aggggtgcattctggaagcc

SEQ ID NO: 11303 - RNA, 20 nt, synthetic construct
  source 1..20: mol_type = other RNA
gactcagaaggggtgcattc

SEQ ID NO: 11304 - RNA, 20 nt, synthetic construct
  source 1..20: mol_type = other RNA
attgagcagggactcagaag

SEQ ID NO: 11305 - RNA, 20 nt, synthetic construct
  source 1..20: mol_type = other RNA
gattgagcagggactcagaa

SEQ ID NO: 11306 - RNA, 20 nt, synthetic construct
  source 1..20: mol_type = other RNA
agattgagcagggactcaga

SEQ ID NO: 11307 - RNA, 20 nt, synthetic construct
  source 1..20: mol_type = other RNA
gaggggtgggagattgagca

SEQ ID NO: 11308 - RNA, 20 nt, synthetic construct
  source 1..20: mol_type = other RNA
tgaggggtgggagattgagc

SEQ ID NO: 11309 - RNA, 20 nt, synthetic construct
  source 1..20: mol_type = other RNA
acccctcattttgctgccct

SEQ ID NO: 11310 - RNA, 20 nt, synthetic construct
  source 1..20: mol_type = other RNA
agggcagcaaaatgaggggt

SEQ ID NO: 11311 - RNA, 20 nt, synthetic construct
  source 1..20: mol_type = other RNA
tagggcagcaaaatgagggg

SEQ ID NO: 11312 - RNA, 20 nt, synthetic construct
  source 1..20: mol_type = other RNA
acctagggcagcaaaatgag

SEQ ID NO: 11313 - RNA, 20 nt, synthetic construct
  source 1..20: mol_type = other RNA
tacctagggcagcaaaatga

SEQ ID NO: 11314 - RNA, 20 nt, synthetic construct
  source 1..20: mol_type = other RNA
atacctagggcagcaaaatg

SEQ ID NO: 11315 - RNA, 20 nt, synthetic construct
  source 1..20: mol_type = other RNA
ctaggtatgccttgatgtcg

SEQ ID NO: 11316 - RNA, 20 nt, synthetic construct
  source 1..20: mol_type = other RNA
gcgacatcaaggcataccta

SEQ ID NO: 11317 - RNA, 20 nt, synthetic construct
  source 1..20: mol_type = other RNA
cgcgacatcaaggcatacct

SEQ ID NO: 11318 - RNA, 20 nt, synthetic construct
  source 1..20: mol_type = other RNA
atgccttgatgtcgcggtgc

SEQ ID NO: 11319 - RNA, 20 nt, synthetic construct
  source 1..20: mol_type = other RNA
tgccttgatgtcgcggtgct

SEQ ID NO: 11320 - RNA, 20 nt, synthetic construct
  source 1..20: mol_type = other RNA
ctcccagcaccgcgacatca

SEQ ID NO: 11321 - RNA, 20 nt, synthetic construct
  source 1..20: mol_type = other RNA
gtgctgggagctaaatcccc

SEQ ID NO: 11322 - RNA, 20 nt, synthetic construct
  source 1..20: mol_type = other RNA
gggagctaaatccccaggac

SEQ ID NO: 11323 - RNA, 20 nt, synthetic construct
  source 1..20: mol_type = other RNA
gtaaaacttggccggtcctg

SEQ ID NO: 11324 - RNA, 20 nt, synthetic construct
  source 1..20: mol_type = other RNA
tgtaaaacttggccggtcct

SEQ ID NO: 11325 - RNA, 20 nt, synthetic construct
  source 1..20: mol_type = other RNA
ctgtaaaacttggccggtcc

SEQ ID NO: 11326 - RNA, 20 nt, synthetic construct
  source 1..20: mol_type = other RNA
ggccaagttttacagagctg

SEQ ID NO: 11327 - RNA, 20 nt, synthetic construct
  source 1..20: mol_type = other RNA
gccaagttttacagagctgc

SEQ ID NO: 11328 - RNA, 20 nt, synthetic construct
  source 1..20: mol_type = other RNA
gcagctctgtaaaacttggc

SEQ ID NO: 11329 - RNA, 20 nt, synthetic construct
  source 1..20: mol_type = other RNA
tcccgcagctctgtaaaact

SEQ ID NO: 11330 - RNA, 20 nt, synthetic construct
  source 1..20: mol_type = other RNA
tacagagctgcgggaagatt

SEQ ID NO: 11331 - RNA, 20 nt, synthetic construct
  source 1..20: mol_type = other RNA
agatttggagaacacactga

SEQ ID NO: 11332 - RNA, 20 nt, synthetic construct
  source 1..20: mol_type = other RNA
gaaggccttgcctcctgccc

SEQ ID NO: 11333 - RNA, 20 nt, synthetic construct
  source 1..20: mol_type = other RNA
aggctcctgggcaggaggca

SEQ ID NO: 11334 - RNA, 20 nt, synthetic construct
  source 1..20: mol_type = other RNA
tcgtcaggctcctgggcagg

SEQ ID NO: 11335 - RNA, 20 nt, synthetic construct
  source 1..20: mol_type = other RNA
atttcgtcaggctcctgggc

SEQ ID NO: 11336 - RNA, 20 nt, synthetic construct
  source 1..20: mol_type = other RNA
gaggatttcgtcaggctcct

SEQ ID NO: 11337 - RNA, 20 nt, synthetic construct
  source 1..20: mol_type = other RNA
agaggatttcgtcaggctcc

SEQ ID NO: 11338 - RNA, 20 nt, synthetic construct
  source 1..20: mol_type = other RNA
ttgacatagaggatttcgtc

SEQ ID NO: 11339 - RNA, 20 nt, synthetic construct
  source 1..20: mol_type = other RNA
cctctatgtcaacatggatg

SEQ ID NO: 11340 - RNA, 20 nt, synthetic construct
  source 1..20: mol_type = other RNA
ctctatgtcaacatggatga

SEQ ID NO: 11341 - RNA, 20 nt, synthetic construct
  source 1..20: mol_type = other RNA
tatgtcaacatggatgaggg

SEQ ID NO: 11342 - RNA, 20 nt, synthetic construct
  source 1..20: mol_type = other RNA
cctcatccatgttgacatag

SEQ ID NO: 11343 - RNA, 20 nt, synthetic construct
  source 1..20: mol_type = other RNA
gtcaacatggatgagggtgg

SEQ ID NO: 11344 - RNA, 20 nt, synthetic construct
  source 1..20: mol_type = other RNA
ggaggttatcctgaaccccc

SEQ ID NO: 11345 - RNA, 20 nt, synthetic construct
  source 1..20: mol_type = other RNA
cctgaaccccctggagctgc

SEQ ID NO: 11346 - RNA, 20 nt, synthetic construct
  source 1..20: mol_type = other RNA
gaaccccctggagctgcagg

SEQ ID NO: 11347 - RNA, 20 nt, synthetic construct
  source 1..20: mol_type = other RNA
cctgcagctccagggggttc

SEQ ID NO: 11348 - RNA, 20 nt, synthetic construct
  source 1..20: mol_type = other RNA
gctcctcctgcagctccagg

SEQ ID NO: 11349 - RNA, 20 nt, synthetic construct
  source 1..20: mol_type = other RNA
agctcctcctgcagctccag

SEQ ID NO: 11350 - RNA, 20 nt, synthetic construct
  source 1..20: mol_type = other RNA
cagctcctcctgcagctcca

SEQ ID NO: 11351 - RNA, 20 nt, synthetic construct
  source 1..20: mol_type = other RNA
tcagctcctcctgcagctcc

SEQ ID NO: 11352 - RNA, 20 nt, synthetic construct
  source 1..20: mol_type = other RNA
cccaacccagccagacccta

SEQ ID NO: 11353 - RNA, 20 nt, synthetic construct
  source 1..20: mol_type = other RNA
tagggtctggctgggttggg

SEQ ID NO: 11354 - RNA, 20 nt, synthetic construct
  source 1..20: mol_type = other RNA
ttagggtctggctgggttgg

SEQ ID NO: 11355 - RNA, 20 nt, synthetic construct
  source 1..20: mol_type = other RNA
cttagggtctggctgggttg

SEQ ID NO: 11356 - RNA, 20 nt, synthetic construct
  source 1..20: mol_type = other RNA
ccttagggtctggctgggtt

SEQ ID NO: 11357 - RNA, 20 nt, synthetic construct
  source 1..20: mol_type = other RNA
tccttagggtctggctgggt

SEQ ID NO: 11358 - RNA, 20 nt, synthetic construct
  source 1..20: mol_type = other RNA
ggaatccttagggtctggct

SEQ ID NO: 11359 - RNA, 20 nt, synthetic construct
  source 1..20: mol_type = other RNA
aggaatccttagggtctggc

SEQ ID NO: 11360 - RNA, 20 nt, synthetic construct
  source 1..20: mol_type = other RNA
ctacaggaatccttagggtc

SEQ ID NO: 11361 - RNA, 20 nt, synthetic construct
  source 1..20: mol_type = other RNA
ggcagctacaggaatcctta

SEQ ID NO: 11362 - RNA, 20 nt, synthetic construct
  source 1..20: mol_type = other RNA
aggcagctacaggaatcctt

SEQ ID NO: 11363 - RNA, 20 nt, synthetic construct
  source 1..20: mol_type = other RNA
ttcctgtagctgcctcactg

SEQ ID NO: 11364 - RNA, 20 nt, synthetic construct
  source 1..20: mol_type = other RNA
tagctgcctcactgcggctg

SEQ ID NO: 11365 - RNA, 20 nt, synthetic construct
  source 1..20: mol_type = other RNA
agccgcagtgaggcagctac

SEQ ID NO: 11366 - RNA, 20 nt, synthetic construct
  source 1..20: mol_type = other RNA
gatggacctcagccgcagtg

SEQ ID NO: 11367 - RNA, 20 nt, synthetic construct
  source 1..20: mol_type = other RNA
gcggctgaggtccatcctgc

SEQ ID NO: 11368 - RNA, 20 nt, synthetic construct
  source 1..20: mol_type = other RNA
ggacatagcgtccagcagga

SEQ ID NO: 11369 - RNA, 20 nt, synthetic construct
  source 1..20: mol_type = other RNA
cagaggacatagcgtccagc

SEQ ID NO: 11370 - RNA, 20 nt, synthetic construct
  source 1..20: mol_type = other RNA
taggggttgtggaagggcag

SEQ ID NO: 11371 - RNA, 20 nt, synthetic construct
  source 1..20: mol_type = other RNA
cggggctaggggttgtggaa

SEQ ID NO: 11372 - RNA, 20 nt, synthetic construct
  source 1..20: mol_type = other RNA
gcggggctaggggttgtgga

SEQ ID NO: 11373 - RNA, 20 nt, synthetic construct
  source 1..20: mol_type = other RNA
ctgagcggggctaggggttg

SEQ ID NO: 11374 - RNA, 20 nt, synthetic construct
  source 1..20: mol_type = other RNA
agcaggctgagcggggctag

SEQ ID NO: 11375 - RNA, 20 nt, synthetic construct
  source 1..20: mol_type = other RNA
cagcaggctgagcggggcta

SEQ ID NO: 11376 - RNA, 20 nt, synthetic construct
  source 1..20: mol_type = other RNA
tcagcaggctgagcggggct

SEQ ID NO: 11377 - RNA, 20 nt, synthetic construct
  source 1..20: mol_type = other RNA
cccgctcagcctgctgatag

SEQ ID NO: 11378 - RNA, 20 nt, synthetic construct
  source 1..20: mol_type = other RNA
ccctatcagcaggctgagcg

SEQ ID NO: 11379 - RNA, 20 nt, synthetic construct
  source 1..20: mol_type = other RNA
cccctatcagcaggctgagc

SEQ ID NO: 11380 - RNA, 20 nt, synthetic construct
  source 1..20: mol_type = other RNA
gcccctatcagcaggctgag

SEQ ID NO: 11381 - RNA, 20 nt, synthetic construct
  source 1..20: mol_type = other RNA
gctggggagcccctatcagc

SEQ ID NO: 11382 - RNA, 20 nt, synthetic construct
  source 1..20: mol_type = other RNA
aggggctccccagcagcccc

SEQ ID NO: 11383 - RNA, 20 nt, synthetic construct
  source 1..20: mol_type = other RNA
ggggctccccagcagcccca

SEQ ID NO: 11384 - RNA, 20 nt, synthetic construct
  source 1..20: mol_type = other RNA
ctccccagcagccccagggc

SEQ ID NO: 11385 - RNA, 20 nt, synthetic construct
  source 1..20: mol_type = other RNA
cccagcagccccagggcagg

SEQ ID NO: 11386 - RNA, 20 nt, synthetic construct
  source 1..20: mol_type = other RNA
ctcctgccctggggctgctg

SEQ ID NO: 11387 - RNA, 20 nt, synthetic construct
  source 1..20: mol_type = other RNA
cctcctgccctggggctgct

SEQ ID NO: 11388 - RNA, 20 nt, synthetic construct
  source 1..20: mol_type = other RNA
tcctcctgccctggggctgc

SEQ ID NO: 11389 - RNA, 20 nt, synthetic construct
  source 1..20: mol_type = other RNA
ggcaccatcctcctgccctg

SEQ ID NO: 11390 - RNA, 20 nt, synthetic construct
  source 1..20: mol_type = other RNA
aggcaccatcctcctgccct

SEQ ID NO: 11391 - RNA, 20 nt, synthetic construct
  source 1..20: mol_type = other RNA
caggcaccatcctcctgccc

SEQ ID NO: 11392 - RNA, 20 nt, synthetic construct
  source 1..20: mol_type = other RNA
gcctgagacaaccctccacc

SEQ ID NO: 11393 - RNA, 20 nt, synthetic construct
  source 1..20: mol_type = other RNA
accaggtggagggttgtctc

SEQ ID NO: 11394 - RNA, 20 nt, synthetic construct
  source 1..20: mol_type = other RNA
tccacctggtactccctctc

SEQ ID NO: 11395 - RNA, 20 nt, synthetic construct
  source 1..20: mol_type = other RNA
gagagggagtaccaggtgga

SEQ ID NO: 11396 - RNA, 20 nt, synthetic construct
  source 1..20: mol_type = other RNA
tgagagggagtaccaggtgg

SEQ ID NO: 11397 - RNA, 20 nt, synthetic construct
  source 1..20: mol_type = other RNA
tcctgagagggagtaccagg

SEQ ID NO: 11398 - RNA, 20 nt, synthetic construct
  source 1..20: mol_type = other RNA
ggatcctgagagggagtacc

SEQ ID NO: 11399 - RNA, 20 nt, synthetic construct
  source 1..20: mol_type = other RNA
gcttagcttggatcctgaga

SEQ ID NO: 11400 - RNA, 20 nt, synthetic construct
  source 1..20: mol_type = other RNA
tgcttagcttggatcctgag

SEQ ID NO: 11401 - RNA, 20 nt, synthetic construct
  source 1..20: mol_type = other RNA
tccaagctaagcactgccac

SEQ ID NO: 11402 - RNA, 20 nt, synthetic construct
  source 1..20: mol_type = other RNA
ccaagctaagcactgccact

SEQ ID NO: 11403 - RNA, 20 nt, synthetic construct
  source 1..20: mol_type = other RNA
caagctaagcactgccactg

SEQ ID NO: 11404 - RNA, 20 nt, synthetic construct
  source 1..20: mol_type = other RNA
cccagtggcagtgcttagct

SEQ ID NO: 11405 - RNA, 20 nt, synthetic construct
  source 1..20: mol_type = other RNA
gaaggtggagttttccccag

SEQ ID NO: 11406 - RNA, 20 nt, synthetic construct
  source 1..20: mol_type = other RNA
ggggtgggaaagtgggaagg

SEQ ID NO: 11407 - RNA, 20 nt, synthetic construct
  source 1..20: mol_type = other RNA
cgtggggtgggaaagtggga

SEQ ID NO: 11408 - RNA, 20 nt, synthetic construct
  source 1..20: mol_type = other RNA
aaggcgtggggtgggaaagt

SEQ ID NO: 11409 - RNA, 20 nt, synthetic construct
  source 1..20: mol_type = other RNA
taaggcgtggggtgggaaag

SEQ ID NO: 11410 - RNA, 20 nt, synthetic construct
  source 1..20: mol_type = other RNA
gtggggataaggcgtggggt

SEQ ID NO: 11411 - RNA, 20 nt, synthetic construct
  source 1..20: mol_type = other RNA
agtggggataaggcgtgggg

SEQ ID NO: 11412 - RNA, 20 nt, synthetic construct
  source 1..20: mol_type = other RNA
gcaagtggggataaggcgtg

SEQ ID NO: 11413 - RNA, 20 nt, synthetic construct
  source 1..20: mol_type = other RNA
tgcaagtggggataaggcgt

SEQ ID NO: 11414 - RNA, 20 nt, synthetic construct
  source 1..20: mol_type = other RNA
ctgcaagtggggataaggcg

SEQ ID NO: 11415 - RNA, 20 nt, synthetic construct
  source 1..20: mol_type = other RNA
cagggctgcaagtggggata

SEQ ID NO: 11416 - RNA, 20 nt, synthetic construct
  source 1..20: mol_type = other RNA
ggaagacagggctgcaagtg

SEQ ID NO: 11417 - RNA, 20 nt, synthetic construct
  source 1..20: mol_type = other RNA
aggaagacagggctgcaagt

SEQ ID NO: 11418 - RNA, 20 nt, synthetic construct
  source 1..20: mol_type = other RNA
taggaagacagggctgcaag

SEQ ID NO: 11419 - RNA, 20 nt, synthetic construct
  source 1..20: mol_type = other RNA
gtgggataggtaggaagaca

SEQ ID NO: 11420 - RNA, 20 nt, synthetic construct
  source 1..20: mol_type = other RNA
ggtgggataggtaggaagac

SEQ ID NO: 11421 - RNA, 20 nt, synthetic construct
  source 1..20: mol_type = other RNA
gggatggaggtgggataggt

SEQ ID NO: 11422 - RNA, 20 nt, synthetic construct
  source 1..20: mol_type = other RNA
atcccacctccatcccagac

SEQ ID NO: 11423 - RNA, 20 nt, synthetic construct
  source 1..20: mol_type = other RNA
gtctgggatggaggtgggat

SEQ ID NO: 11424 - RNA, 20 nt, synthetic construct
  source 1..20: mol_type = other RNA
gacctgtctgggatggaggt

SEQ ID NO: 11425 - RNA, 20 nt, synthetic construct
  source 1..20: mol_type = other RNA
ggacctgtctgggatggagg

SEQ ID NO: 11426 - RNA, 20 nt, synthetic construct
  source 1..20: mol_type = other RNA
gagggacctgtctgggatgg

SEQ ID NO: 11427 - RNA, 20 nt, synthetic construct
  source 1..20: mol_type = other RNA
ggggagggacctgtctggga

SEQ ID NO: 11428 - RNA, 20 nt, synthetic construct
  source 1..20: mol_type = other RNA
agaaggggagggacctgtct

SEQ ID NO: 11429 - RNA, 20 nt, synthetic construct
  source 1..20: mol_type = other RNA
gagaaggggagggacctgtc

SEQ ID NO: 11430 - RNA, 20 nt, synthetic construct
  source 1..20: mol_type = other RNA
ctactgcacagagaagggga

SEQ ID NO: 11431 - RNA, 20 nt, synthetic construct
  source 1..20: mol_type = other RNA
gctactgcacagagaagggg

SEQ ID NO: 11432 - RNA, 20 nt, synthetic construct
  source 1..20: mol_type = other RNA
gatgctactgcacagagaag

SEQ ID NO: 11433 - RNA, 20 nt, synthetic construct
  source 1..20: mol_type = other RNA
tgatgctactgcacagagaa

SEQ ID NO: 11434 - RNA, 20 nt, synthetic construct
  source 1..20: mol_type = other RNA
gtgatgctactgcacagaga

SEQ ID NO: 11435 - RNA, 20 nt, synthetic construct
  source 1..20: mol_type = other RNA
tggtgatgctactgctttca

SEQ ID NO: 11436 - RNA, 20 nt, synthetic construct
  source 1..20: mol_type = other RNA
gtagcatcaccatctgtaaa

SEQ ID NO: 11437 - RNA, 20 nt, synthetic construct
  source 1..20: mol_type = other RNA
catcaccatctgtaaaagga

SEQ ID NO: 11438 - RNA, 20 nt, synthetic construct
  source 1..20: mol_type = other RNA
atcaccatctgtaaaaggaa

SEQ ID NO: 11439 - RNA, 20 nt, synthetic construct
  source 1..20: mol_type = other RNA
tcaccatctgtaaaaggaag

SEQ ID NO: 11440 - RNA, 20 nt, synthetic construct
  source 1..20: mol_type = other RNA
catctgtaaaaggaaggggt

SEQ ID NO: 11441 - RNA, 20 nt, synthetic construct
  source 1..20: mol_type = other RNA
caaccccttccttttacaga

SEQ ID NO: 11442 - RNA, 20 nt, synthetic construct
  source 1..20: mol_type = other RNA
gcaatatctgaagccctccc

SEQ ID NO: 11443 - RNA, 20 nt, synthetic construct
  source 1..20: mol_type = other RNA
tggaatgttaacacctggga

SEQ ID NO: 11444 - RNA, 20 nt, synthetic construct
  source 1..20: mol_type = other RNA
ttggaatgttaacacctggg

SEQ ID NO: 11445 - RNA, 20 nt, synthetic construct
  source 1..20: mol_type = other RNA
gtcttggaatgttaacacct

SEQ ID NO: 11446 - RNA, 20 nt, synthetic construct
  source 1..20: mol_type = other RNA
agtcttggaatgttaacacc

SEQ ID NO: 11447 - RNA, 20 nt, synthetic construct
  source 1..20: mol_type = other RNA
ttccaagactctagagtcca

SEQ ID NO: 11448 - RNA, 20 nt, synthetic construct
  source 1..20: mol_type = other RNA
aaccttggactctagagtct

SEQ ID NO: 11449 - RNA, 20 nt, synthetic construct
  source 1..20: mol_type = other RNA
aatctagactctttaaacct

SEQ ID NO: 11450 - RNA, 20 nt, synthetic construct
  source 1..20: mol_type = other RNA
tttaaagagtctagattcaa

SEQ ID NO: 11451 - RNA, 20 nt, synthetic construct
  source 1..20: mol_type = other RNA
agtctagattcaaaggttct

SEQ ID NO: 11452 - RNA, 20 nt, synthetic construct
  source 1..20: mol_type = other RNA
tcaaagatgctgtgagtctt

SEQ ID NO: 11453 - RNA, 20 nt, synthetic construct
  source 1..20: mol_type = other RNA
gctgtgagtctttggttcta

SEQ ID NO: 11454 - RNA, 20 nt, synthetic construct
  source 1..20: mol_type = other RNA
attagagactttggaatttc

SEQ ID NO: 11455 - RNA, 20 nt, synthetic construct
  source 1..20: mol_type = other RNA
tttaatagaattagagactt

SEQ ID NO: 11456 - RNA, 20 nt, synthetic construct
  source 1..20: mol_type = other RNA
ctaattctattaaagtgcta

SEQ ID NO: 11457 - RNA, 20 nt, synthetic construct
  source 1..20: mol_type = other RNA
attaaagtgctaaggttcta

SEQ ID NO: 11458 - RNA, 20 nt, synthetic construct
  source 1..20: mol_type = other RNA
aaaaaaaaaaaaaaaaaagt

SEQ ID NO: 11459 - RNA, 20 nt, synthetic construct
  source 1..20: mol_type = other RNA
agagtctcactgtgtcaccc

SEQ ID NO: 11460 - RNA, 20 nt, synthetic construct
  source 1..20: mol_type = other RNA
tctcactgtgtcacccaggc

SEQ ID NO: 11461 - RNA, 20 nt, synthetic construct
  source 1..20: mol_type = other RNA
tcacccaggctggagtgcag

SEQ ID NO: 11462 - RNA, 20 nt, synthetic construct
  source 1..20: mol_type = other RNA
gcaccactgcactccagcct

SEQ ID NO: 11463 - RNA, 20 nt, synthetic construct
  source 1..20: mol_type = other RNA
tgcaccactgcactccagcc

SEQ ID NO: 11464 - RNA, 20 nt, synthetic construct
  source 1..20: mol_type = other RNA
ggtaggtgaaggttgcagtg

SEQ ID NO: 11465 - RNA, 20 nt, synthetic construct
  source 1..20: mol_type = other RNA
cacttgaactcggtaggtga

SEQ ID NO: 11466 - RNA, 20 nt, synthetic construct
  source 1..20: mol_type = other RNA
gaaaatcacttgaactcggt

SEQ ID NO: 11467 - RNA, 20 nt, synthetic construct
  source 1..20: mol_type = other RNA
ttcaagtgattttcctgcct

SEQ ID NO: 11468 - RNA, 20 nt, synthetic construct
  source 1..20: mol_type = other RNA
gccttggcctcccaagtagc

SEQ ID NO: 11469 - RNA, 20 nt, synthetic construct
  source 1..20: mol_type = other RNA
ccttggcctcccaagtagct

SEQ ID NO: 11470 - RNA, 20 nt, synthetic construct
  source 1..20: mol_type = other RNA
gctacttgggaggccaaggc

SEQ ID NO: 11471 - RNA, 20 nt, synthetic construct
  source 1..20: mol_type = other RNA
cccagctacttgggaggcca

SEQ ID NO: 11472 - RNA, 20 nt, synthetic construct
  source 1..20: mol_type = other RNA
tcccaagtagctgggattac

SEQ ID NO: 11473 - RNA, 20 nt, synthetic construct
  source 1..20: mol_type = other RNA
tgtaatcccagctacttggg

SEQ ID NO: 11474 - RNA, 20 nt, synthetic construct
  source 1..20: mol_type = other RNA
acctgtaatcccagctactt

SEQ ID NO: 11475 - RNA, 20 nt, synthetic construct
  source 1..20: mol_type = other RNA
cacctgtaatcccagctact

SEQ ID NO: 11476 - RNA, 20 nt, synthetic construct
  source 1..20: mol_type = other RNA
caggtgtgtgccaccacacc

SEQ ID NO: 11477 - RNA, 20 nt, synthetic construct
  source 1..20: mol_type = other RNA
taaaaattagccgggtgtgg

SEQ ID NO: 11478 - RNA, 20 nt, synthetic construct
  source 1..20: mol_type = other RNA
atataaaaattagccgggtg

SEQ ID NO: 11479 - RNA, 20 nt, synthetic construct
  source 1..20: mol_type = other RNA
taaaaatataaaaattagcc

SEQ ID NO: 11480 - RNA, 20 nt, synthetic construct
  source 1..20: mol_type = other RNA
ctaaaaatataaaaattagc

SEQ ID NO: 11481 - RNA, 20 nt, synthetic construct
  source 1..20: mol_type = other RNA
tttatatttttagtagagac

SEQ ID NO: 11482 - RNA, 20 nt, synthetic construct
  source 1..20: mol_type = other RNA
ttatatttttagtagagaca

SEQ ID NO: 11483 - RNA, 20 nt, synthetic construct
  source 1..20: mol_type = other RNA
gagacagggtttcaccatgt

SEQ ID NO: 11484 - RNA, 20 nt, synthetic construct
  source 1..20: mol_type = other RNA
agggtttcaccatgttggcc

SEQ ID NO: 11485 - RNA, 20 nt, synthetic construct
  source 1..20: mol_type = other RNA
tttcaccatgttggccaggc

SEQ ID NO: 11486 - RNA, 20 nt, synthetic construct
  source 1..20: mol_type = other RNA
ttagaccagcctggccaaca

SEQ ID NO: 11487 - RNA, 20 nt, synthetic construct
  source 1..20: mol_type = other RNA
tcaggagttttagaccagcc

SEQ ID NO: 11488 - RNA, 20 nt, synthetic construct
  source 1..20: mol_type = other RNA
tgggcagatcacttgaggtc

SEQ ID NO: 11489 - RNA, 20 nt, synthetic construct
  source 1..20: mol_type = other RNA
tgaggtgggcagatcacttg

SEQ ID NO: 11490 - RNA, 20 nt, synthetic construct
  source 1..20: mol_type = other RNA
gcactttgggaggctgaggt

SEQ ID NO: 11491 - RNA, 20 nt, synthetic construct
  source 1..20: mol_type = other RNA
agcactttgggaggctgagg

SEQ ID NO: 11492 - RNA, 20 nt, synthetic construct
  source 1..20: mol_type = other RNA
ctcagcactttgggaggctg

SEQ ID NO: 11493 - RNA, 20 nt, synthetic construct
  source 1..20: mol_type = other RNA
tcccaaagtgctgagattac

SEQ ID NO: 11494 - RNA, 20 nt, synthetic construct
  source 1..20: mol_type = other RNA
tgtaatctcagcactttggg

SEQ ID NO: 11495 - RNA, 20 nt, synthetic construct
  source 1..20: mol_type = other RNA
gcctgtaatctcagcacttt

SEQ ID NO: 11496 - RNA, 20 nt, synthetic construct
  source 1..20: mol_type = other RNA
tgcctgtaatctcagcactt

SEQ ID NO: 11497 - RNA, 20 nt, synthetic construct
  source 1..20: mol_type = other RNA
ggtcttaaggttgagtgcag

SEQ ID NO: 11498 - RNA, 20 nt, synthetic construct
  source 1..20: mol_type = other RNA
ctttagaacagtaggtctta

SEQ ID NO: 11499 - RNA, 20 nt, synthetic construct
  source 1..20: mol_type = other RNA
tgtcagagctttagaacagt

SEQ ID NO: 11500 - RNA, 20 nt, synthetic construct
  source 1..20: mol_type = other RNA
tctaaagctctgacattatg

SEQ ID NO: 11501 - RNA, 20 nt, synthetic construct
  source 1..20: mol_type = other RNA
ttatgtggttttagattttc

SEQ ID NO: 11502 - RNA, 20 nt, synthetic construct
  source 1..20: mol_type = other RNA
acatttttgataaagcctca

SEQ ID NO: 11503 - RNA, 20 nt, synthetic construct
  source 1..20: mol_type = other RNA
tgataaagcctcaaggtttt

SEQ ID NO: 11504 - RNA, 20 nt, synthetic construct
  source 1..20: mol_type = other RNA
ctttagaacctaaaaccttg

SEQ ID NO: 11505 - RNA, 20 nt, synthetic construct
  source 1..20: mol_type = other RNA
agttctaagattctgatttt

SEQ ID NO: 11506 - RNA, 20 nt, synthetic construct
  source 1..20: mol_type = other RNA
gattctgattttaggagcta

SEQ ID NO: 11507 - RNA, 20 nt, synthetic construct
  source 1..20: mol_type = other RNA
atctataatcttacatttta

SEQ ID NO: 11508 - RNA, 20 nt, synthetic construct
  source 1..20: mol_type = other RNA
agattctatagttctagaca

SEQ ID NO: 11509 - RNA, 20 nt, synthetic construct
  source 1..20: mol_type = other RNA
ttctatagttctagacatgg

SEQ ID NO: 11510 - RNA, 20 nt, synthetic construct
  source 1..20: mol_type = other RNA
ttctagacatggaggttcta

SEQ ID NO: 11511 - RNA, 20 nt, synthetic construct
  source 1..20: mol_type = other RNA
acatggaggttctaaggcct

SEQ ID NO: 11512 - RNA, 20 nt, synthetic construct
  source 1..20: mol_type = other RNA
acatcacattttagaatcct

SEQ ID NO: 11513 - RNA, 20 nt, synthetic construct
  source 1..20: mol_type = other RNA
ttctaaaatgtgatgttcta

SEQ ID NO: 11514 - RNA, 20 nt, synthetic construct
  source 1..20: mol_type = other RNA
ctctgagagtctagattctc

SEQ ID NO: 11515 - RNA, 20 nt, synthetic construct
  source 1..20: mol_type = other RNA
gtctagattctctggctgta

SEQ ID NO: 11516 - RNA, 20 nt, synthetic construct
  source 1..20: mol_type = other RNA
ctgtaaggctctagatcata

SEQ ID NO: 11517 - RNA, 20 nt, synthetic construct
  source 1..20: mol_type = other RNA
atgatcaattatagtttctg

SEQ ID NO: 11518 - RNA, 20 nt, synthetic construct
  source 1..20: mol_type = other RNA
gtataagatcctagatccta

SEQ ID NO: 11519 - RNA, 20 nt, synthetic construct
  source 1..20: mol_type = other RNA
tataagatcctagatcctaa

SEQ ID NO: 11520 - RNA, 20 nt, synthetic construct
  source 1..20: mol_type = other RNA
gctttcgacccttaggatct

SEQ ID NO: 11521 - RNA, 20 nt, synthetic construct
  source 1..20: mol_type = other RNA
ttctagagctttcgaccctt

SEQ ID NO: 11522 - RNA, 20 nt, synthetic construct
  source 1..20: mol_type = other RNA
aagttccaagagtctaaaga

SEQ ID NO: 11523 - RNA, 20 nt, synthetic construct
  source 1..20: mol_type = other RNA
aaactccatctttagactct

SEQ ID NO: 11524 - RNA, 20 nt, synthetic construct
  source 1..20: mol_type = other RNA
gtctaaagatggagtttcta

SEQ ID NO: 11525 - RNA, 20 nt, synthetic construct
  source 1..20: mol_type = other RNA
aagatggagtttctaaggtc

SEQ ID NO: 11526 - RNA, 20 nt, synthetic construct
  source 1..20: mol_type = other RNA
aatatcacatcttagaacac

SEQ ID NO: 11527 - RNA, 20 nt, synthetic construct
  source 1..20: mol_type = other RNA
tatttaatcatctagaatct

SEQ ID NO: 11528 - RNA, 20 nt, synthetic construct
  source 1..20: mol_type = other RNA
atgattaaataagattctaa

SEQ ID NO: 11529 - RNA, 20 nt, synthetic construct
  source 1..20: mol_type = other RNA
taacggtctgttctgtttca

SEQ ID NO: 11530 - RNA, 20 nt, synthetic construct
  source 1..20: mol_type = other RNA
caaggcactctagattccat

SEQ ID NO: 11531 - RNA, 20 nt, synthetic construct
  source 1..20: mol_type = other RNA
attccattggtccaagattc

SEQ ID NO: 11532 - RNA, 20 nt, synthetic construct
  source 1..20: mol_type = other RNA
gatccggaatcttggaccaa

SEQ ID NO: 11533 - RNA, 20 nt, synthetic construct
  source 1..20: mol_type = other RNA
atgcttaggatccggaatct

SEQ ID NO: 11534 - RNA, 20 nt, synthetic construct
  source 1..20: mol_type = other RNA
taacttagatgcttaggatc

SEQ ID NO: 11535 - RNA, 20 nt, synthetic construct
  source 1..20: mol_type = other RNA
gtcttataacttagatgctt

SEQ ID NO: 11536 - RNA, 20 nt, synthetic construct
  source 1..20: mol_type = other RNA
attagaaattattagaactt

SEQ ID NO: 11537 - RNA, 20 nt, synthetic construct
  source 1..20: mol_type = other RNA
ttctaatgttggacaccttt

SEQ ID NO: 11538 - RNA, 20 nt, synthetic construct
  source 1..20: mol_type = other RNA
gaatgcagcaaagaacctaa

SEQ ID NO: 11539 - RNA, 20 nt, synthetic construct
  source 1..20: mol_type = other RNA
ttgctgcattctgcctctct

SEQ ID NO: 11540 - RNA, 20 nt, synthetic construct
  source 1..20: mol_type = other RNA
attctgcctctctaggacca

SEQ ID NO: 11541 - RNA, 20 nt, synthetic construct
  source 1..20: mol_type = other RNA
tcttaaccatggtcctagag

SEQ ID NO: 11542 - RNA, 20 nt, synthetic construct
  source 1..20: mol_type = other RNA
gattcttggactcttaacca

SEQ ID NO: 11543 - RNA, 20 nt, synthetic construct
  source 1..20: mol_type = other RNA
attttagaaatgtggattct

SEQ ID NO: 11544 - RNA, 20 nt, synthetic construct
  source 1..20: mol_type = other RNA
actataagattttagaaatg

SEQ ID NO: 11545 - RNA, 20 nt, synthetic construct
  source 1..20: mol_type = other RNA
ttctaaaatcttatagttct

SEQ ID NO: 11546 - RNA, 20 nt, synthetic construct
  source 1..20: mol_type = other RNA
ctaagtttctaagattctaa

SEQ ID NO: 11547 - RNA, 20 nt, synthetic construct
  source 1..20: mol_type = other RNA
ctaagattctaaaggtccac

SEQ ID NO: 11548 - RNA, 20 nt, synthetic construct
  source 1..20: mol_type = other RNA
gtccacaggtctagactatt

SEQ ID NO: 11549 - RNA, 20 nt, synthetic construct
  source 1..20: mol_type = other RNA
cacctaatagtctagacctg

SEQ ID NO: 11550 - RNA, 20 nt, synthetic construct
  source 1..20: mol_type = other RNA
gactattaggtgcaatttca

SEQ ID NO: 11551 - RNA, 20 nt, synthetic construct
  source 1..20: mol_type = other RNA
ccctatactgtagtattctt

SEQ ID NO: 11552 - RNA, 20 nt, synthetic construct
  source 1..20: mol_type = other RNA
cctatactgtagtattcttt

SEQ ID NO: 11553 - RNA, 20 nt, synthetic construct
  source 1..20: mol_type = other RNA
ctatactgtagtattctttg

SEQ ID NO: 11554 - RNA, 20 nt, synthetic construct
  source 1..20: mol_type = other RNA
ccaaagaatactacagtata

SEQ ID NO: 11555 - RNA, 20 nt, synthetic construct
  source 1..20: mol_type = other RNA
cccaaagaatactacagtat

SEQ ID NO: 11556 - RNA, 20 nt, synthetic construct
  source 1..20: mol_type = other RNA
atgatagctaagaaggagag

SEQ ID NO: 11557 - RNA, 20 nt, synthetic construct
  source 1..20: mol_type = other RNA
aatgatagctaagaaggaga

SEQ ID NO: 11558 - RNA, 20 nt, synthetic construct
  source 1..20: mol_type = other RNA
caatgatagctaagaaggag

SEQ ID NO: 11559 - RNA, 20 nt, synthetic construct
  source 1..20: mol_type = other RNA
ggaagcaatgatagctaaga

SEQ ID NO: 11560 - RNA, 20 nt, synthetic construct
  source 1..20: mol_type = other RNA
tgcttcctcctccccaactg

SEQ ID NO: 11561 - RNA, 20 nt, synthetic construct
  source 1..20: mol_type = other RNA
gcttcctcctccccaactgt

SEQ ID NO: 11562 - RNA, 20 nt, synthetic construct
  source 1..20: mol_type = other RNA
cttcctcctccccaactgtg

SEQ ID NO: 11563 - RNA, 20 nt, synthetic construct
  source 1..20: mol_type = other RNA
ttcctcctccccaactgtgg

SEQ ID NO: 11564 - RNA, 20 nt, synthetic construct
  source 1..20: mol_type = other RNA
cacccccacagttggggagg

SEQ ID NO: 11565 - RNA, 20 nt, synthetic construct
  source 1..20: mol_type = other RNA
gcacacccccacagttgggg

SEQ ID NO: 11566 - RNA, 20 nt, synthetic construct
  source 1..20: mol_type = other RNA
ggggcacacccccacagttg

SEQ ID NO: 11567 - RNA, 20 nt, synthetic construct
  source 1..20: mol_type = other RNA
gggggcacacccccacagtt

SEQ ID NO: 11568 - RNA, 20 nt, synthetic construct
  source 1..20: mol_type = other RNA
agggggcacacccccacagt

SEQ ID NO: 11569 - RNA, 20 nt, synthetic construct
  source 1..20: mol_type = other RNA
gcattgcacaggcttgaagg

SEQ ID NO: 11570 - RNA, 20 nt, synthetic construct
  source 1..20: mol_type = other RNA
tcaagcctgtgcaatgcatt

SEQ ID NO: 11571 - RNA, 20 nt, synthetic construct
  source 1..20: mol_type = other RNA
caagcctgtgcaatgcatta

SEQ ID NO: 11572 - RNA, 20 nt, synthetic construct
  source 1..20: mol_type = other RNA
aatgcattgcacaggcttga

SEQ ID NO: 11573 - RNA, 20 nt, synthetic construct
  source 1..20: mol_type = other RNA
gcatccctaatgcattgcac

SEQ ID NO: 11574 - RNA, 20 nt, synthetic construct
  source 1..20: mol_type = other RNA
agggatgcctcctttcccgc

SEQ ID NO: 11575 - RNA, 20 nt, synthetic construct
  source 1..20: mol_type = other RNA
gggatgcctcctttcccgca

SEQ ID NO: 11576 - RNA, 20 nt, synthetic construct
  source 1..20: mol_type = other RNA
ggatgcctcctttcccgcag

SEQ ID NO: 11577 - RNA, 20 nt, synthetic construct
  source 1..20: mol_type = other RNA
gcctcctttcccgcagggga

SEQ ID NO: 11578 - RNA, 20 nt, synthetic construct
  source 1..20: mol_type = other RNA
tccatcccctgcgggaaagg

SEQ ID NO: 11579 - RNA, 20 nt, synthetic construct
  source 1..20: mol_type = other RNA
tcgtccatcccctgcgggaa

SEQ ID NO: 11580 - RNA, 20 nt, synthetic construct
  source 1..20: mol_type = other RNA
ggagatcgtccatcccctgc

SEQ ID NO: 11581 - RNA, 20 nt, synthetic construct
  source 1..20: mol_type = other RNA
gggagatcgtccatcccctg

SEQ ID NO: 11582 - RNA, 20 nt, synthetic construct
  source 1..20: mol_type = other RNA
atggacgatctcccaccttt

SEQ ID NO: 11583 - RNA, 20 nt, synthetic construct
  source 1..20: mol_type = other RNA
tggacgatctcccacctttc

SEQ ID NO: 11584 - RNA, 20 nt, synthetic construct
  source 1..20: mol_type = other RNA
ggcaacatggcccgaaaggt

SEQ ID NO: 11585 - RNA, 20 nt, synthetic construct
  source 1..20: mol_type = other RNA
gggcaacatggcccgaaagg

SEQ ID NO: 11586 - RNA, 20 nt, synthetic construct
  source 1..20: mol_type = other RNA
cgggggcaacatggcccgaa

SEQ ID NO: 11587 - RNA, 20 nt, synthetic construct
  source 1..20: mol_type = other RNA
attggctcacgggggcaaca

SEQ ID NO: 11588 - RNA, 20 nt, synthetic construct
  source 1..20: mol_type = other RNA
ggtgagggattggctcacgg

SEQ ID NO: 11589 - RNA, 20 nt, synthetic construct
  source 1..20: mol_type = other RNA
aggtgagggattggctcacg

SEQ ID NO: 11590 - RNA, 20 nt, synthetic construct
  source 1..20: mol_type = other RNA
aaggtgagggattggctcac

SEQ ID NO: 11591 - RNA, 20 nt, synthetic construct
  source 1..20: mol_type = other RNA
gaaggtgagggattggctca

SEQ ID NO: 11592 - RNA, 20 nt, synthetic construct
  source 1..20: mol_type = other RNA
gtactcagaaggtgagggat

SEQ ID NO: 11593 - RNA, 20 nt, synthetic construct
  source 1..20: mol_type = other RNA
caccttctgagtacagagtg

SEQ ID NO: 11594 - RNA, 20 nt, synthetic construct
  source 1..20: mol_type = other RNA
actctgtactcagaaggtga

SEQ ID NO: 11595 - RNA, 20 nt, synthetic construct
  source 1..20: mol_type = other RNA
cactctgtactcagaaggtg

SEQ ID NO: 11596 - RNA, 20 nt, synthetic construct
  source 1..20: mol_type = other RNA
gtccacactctgtactcaga

SEQ ID NO: 11597 - RNA, 20 nt, synthetic construct
  source 1..20: mol_type = other RNA
gtggactctggtgcctccag

SEQ ID NO: 11598 - RNA, 20 nt, synthetic construct
  source 1..20: mol_type = other RNA
tggactctggtgcctccaga

SEQ ID NO: 11599 - RNA, 20 nt, synthetic construct
  source 1..20: mol_type = other RNA
ggactctggtgcctccagag

SEQ ID NO: 11600 - RNA, 20 nt, synthetic construct
  source 1..20: mol_type = other RNA
tggtgcctccagaggggctc

SEQ ID NO: 11601 - RNA, 20 nt, synthetic construct
  source 1..20: mol_type = other RNA
tgtgacctgagcccctctgg

SEQ ID NO: 11602 - RNA, 20 nt, synthetic construct
  source 1..20: mol_type = other RNA
ttatgtgacctgagcccctc

SEQ ID NO: 11603 - RNA, 20 nt, synthetic construct
  source 1..20: mol_type = other RNA
tcctcatgttgtttatactc

SEQ ID NO: 11604 - RNA, 20 nt, synthetic construct
  source 1..20: mol_type = other RNA
acctgagtataaacaacatg

SEQ ID NO: 11605 - RNA, 20 nt, synthetic construct
  source 1..20: mol_type = other RNA
gtttatactcaggtatttat

SEQ ID NO: 11606 - RNA, 20 nt, synthetic construct
  source 1..20: mol_type = other RNA
tttatactcaggtatttatt

SEQ ID NO: 11607 - RNA, 20 nt, synthetic construct
  source 1..20: mol_type = other RNA
cgtcagtagtccctgataaa

SEQ ID NO: 11608 - RNA, 20 nt, synthetic construct
  source 1..20: mol_type = other RNA
agcgatctttccatttatca

SEQ ID NO: 11609 - RNA, 20 nt, synthetic construct
  source 1..20: mol_type = other RNA
aagcgatctttccatttatc

SEQ ID NO: 11610 - RNA, 20 nt, synthetic construct
  source 1..20: mol_type = other RNA
tggaaagatcgcttgagtcc

SEQ ID NO: 11611 - RNA, 20 nt, synthetic construct
  source 1..20: mol_type = other RNA
ctaggctggactggaactcc

SEQ ID NO: 11612 - RNA, 20 nt, synthetic construct
  source 1..20: mol_type = other RNA
gttccagtccagcctagaat

SEQ ID NO: 11613 - RNA, 20 nt, synthetic construct
  source 1..20: mol_type = other RNA
ttacctattctaggctggac

SEQ ID NO: 11614 - RNA, 20 nt, synthetic construct
  source 1..20: mol_type = other RNA
atgttttacctattctaggc

SEQ ID NO: 11615 - RNA, 20 nt, synthetic construct
  source 1..20: mol_type = other RNA
gagcatgttttacctattct

SEQ ID NO: 11616 - RNA, 20 nt, synthetic construct
  source 1..20: mol_type = other RNA
tctgaattagtctttgaaac

SEQ ID NO: 11617 - RNA, 20 nt, synthetic construct
  source 1..20: mol_type = other RNA
ttttttaagaattccatgag

SEQ ID NO: 11618 - RNA, 20 nt, synthetic construct
  source 1..20: mol_type = other RNA
gaattccatgagtggtttgc

SEQ ID NO: 11619 - RNA, 20 nt, synthetic construct
  source 1..20: mol_type = other RNA
gtacaccagcaaaccactca

SEQ ID NO: 11620 - RNA, 20 nt, synthetic construct
  source 1..20: mol_type = other RNA
gttaggggcttaatttgggg

SEQ ID NO: 11621 - RNA, 20 nt, synthetic construct
  source 1..20: mol_type = other RNA
cgagttaggggcttaatttg

SEQ ID NO: 11622 - RNA, 20 nt, synthetic construct
  source 1..20: mol_type = other RNA
gcgagttaggggcttaattt

SEQ ID NO: 11623 - RNA, 20 nt, synthetic construct
  source 1..20: mol_type = other RNA
tgcgagttaggggcttaatt

SEQ ID NO: 11624 - RNA, 20 nt, synthetic construct
  source 1..20: mol_type = other RNA
cctaactcgcaagcacaaaa

SEQ ID NO: 11625 - RNA, 20 nt, synthetic construct
  source 1..20: mol_type = other RNA
attttgtgcttgcgagttag

SEQ ID NO: 11626 - RNA, 20 nt, synthetic construct
  source 1..20: mol_type = other RNA
cattttgtgcttgcgagtta

SEQ ID NO: 11627 - RNA, 20 nt, synthetic construct
  source 1..20: mol_type = other RNA
ccattttgtgcttgcgagtt

SEQ ID NO: 11628 - RNA, 20 nt, synthetic construct
  source 1..20: mol_type = other RNA
ttatttactgagttatcagt

SEQ ID NO: 11629 - RNA, 20 nt, synthetic construct
  source 1..20: mol_type = other RNA
ggccttgtccttagttgtac

SEQ ID NO: 11630 - RNA, 20 nt, synthetic construct
  source 1..20: mol_type = other RNA
gccttgtccttagttgtaca

SEQ ID NO: 11631 - RNA, 20 nt, synthetic construct
  source 1..20: mol_type = other RNA
tccctgtacaactaaggaca

SEQ ID NO: 11632 - RNA, 20 nt, synthetic construct
  source 1..20: mol_type = other RNA
cattagtccctgtacaacta

SEQ ID NO: 11633 - RNA, 20 nt, synthetic construct
  source 1..20: mol_type = other RNA
aatgactcacctataaataa

SEQ ID NO: 11634 - RNA, 20 nt, synthetic construct
  source 1..20: mol_type = other RNA
atgactcacctataaataat

SEQ ID NO: 11635 - RNA, 20 nt, synthetic construct
  source 1..20: mol_type = other RNA
tagaagagcccattatttat

SEQ ID NO: 11636 - RNA, 20 nt, synthetic construct
  source 1..20: mol_type = other RNA
acacctctttgtcctatagc

SEQ ID NO: 11637 - RNA, 20 nt, synthetic construct
  source 1..20: mol_type = other RNA
cacctctttgtcctatagct

SEQ ID NO: 11638 - RNA, 20 nt, synthetic construct
  source 1..20: mol_type = other RNA
ctctttgtcctatagctggg

SEQ ID NO: 11639 - RNA, 20 nt, synthetic construct
  source 1..20: mol_type = other RNA
ctcccagctataggacaaag

SEQ ID NO: 11640 - RNA, 20 nt, synthetic construct
  source 1..20: mol_type = other RNA
aatgcgttcctcccagctat

SEQ ID NO: 11641 - RNA, 20 nt, synthetic construct
  source 1..20: mol_type = other RNA
caacccaatgattccctaaa

SEQ ID NO: 11642 - RNA, 20 nt, synthetic construct
  source 1..20: mol_type = other RNA
aacccaatgattccctaaat

SEQ ID NO: 11643 - RNA, 20 nt, synthetic construct
  source 1..20: mol_type = other RNA
acccaatgattccctaaatg

SEQ ID NO: 11644 - RNA, 20 nt, synthetic construct
  source 1..20: mol_type = other RNA
catttagggaatcattgggt

SEQ ID NO: 11645 - RNA, 20 nt, synthetic construct
  source 1..20: mol_type = other RNA
accccatttagggaatcatt

SEQ ID NO: 11646 - RNA, 20 nt, synthetic construct
  source 1..20: mol_type = other RNA
gaccccatttagggaatcat

SEQ ID NO: 11647 - RNA, 20 nt, synthetic construct
  source 1..20: mol_type = other RNA
tgatgcgaagaccccattta

SEQ ID NO: 11648 - RNA, 20 nt, synthetic construct
  source 1..20: mol_type = other RNA
ctgatgcgaagaccccattt

SEQ ID NO: 11649 - RNA, 20 nt, synthetic construct
  source 1..20: mol_type = other RNA
tgcgttaaaatcaccccagc

SEQ ID NO: 11650 - RNA, 20 nt, synthetic construct
  source 1..20: mol_type = other RNA
ttaaaatcaccccagcaggc

SEQ ID NO: 11651 - RNA, 20 nt, synthetic construct
  source 1..20: mol_type = other RNA
accccagcaggcaggttatc

SEQ ID NO: 11652 - RNA, 20 nt, synthetic construct
  source 1..20: mol_type = other RNA
gccggataacctgcctgctg

SEQ ID NO: 11653 - RNA, 20 nt, synthetic construct
  source 1..20: mol_type = other RNA
ggccggataacctgcctgct

SEQ ID NO: 11654 - RNA, 20 nt, synthetic construct
  source 1..20: mol_type = other RNA
cggccggataacctgcctgc

SEQ ID NO: 11655 - RNA, 20 nt, synthetic construct
  source 1..20: mol_type = other RNA
ggttatccggccgccactcc

SEQ ID NO: 11656 - RNA, 20 nt, synthetic construct
  source 1..20: mol_type = other RNA
gttatccggccgccactcca

SEQ ID NO: 11657 - RNA, 20 nt, synthetic construct
  source 1..20: mol_type = other RNA
aatgaccctggagtggcggc

SEQ ID NO: 11658 - RNA, 20 nt, synthetic construct
  source 1..20: mol_type = other RNA
atttaatgaccctggagtgg

SEQ ID NO: 11659 - RNA, 20 nt, synthetic construct
  source 1..20: mol_type = other RNA
ctgatttaatgaccctggag

SEQ ID NO: 11660 - RNA, 20 nt, synthetic construct
  source 1..20: mol_type = other RNA
agagtctgatttaatgaccc

SEQ ID NO: 11661 - RNA, 20 nt, synthetic construct
  source 1..20: mol_type = other RNA
cattaaatcagactctccag

SEQ ID NO: 11662 - RNA, 20 nt, synthetic construct
  source 1..20: mol_type = other RNA
attaaatcagactctccagt

SEQ ID NO: 11663 - RNA, 20 nt, synthetic construct
  source 1..20: mol_type = other RNA
cagactctccagtgggacct

SEQ ID NO: 11664 - RNA, 20 nt, synthetic construct
  source 1..20: mol_type = other RNA
tacgaattccgaggtcccac

SEQ ID NO: 11665 - RNA, 20 nt, synthetic construct
  source 1..20: mol_type = other RNA
ttgctaagctacgaattccg

SEQ ID NO: 11666 - RNA, 20 nt, synthetic construct
  source 1..20: mol_type = other RNA
gcaagctccccaagtgatgc

SEQ ID NO: 11667 - RNA, 20 nt, synthetic construct
  source 1..20: mol_type = other RNA
caagctccccaagtgatgct

SEQ ID NO: 11668 - RNA, 20 nt, synthetic construct
  source 1..20: mol_type = other RNA
tttactcccagcatcacttg

SEQ ID NO: 11669 - RNA, 20 nt, synthetic construct
  source 1..20: mol_type = other RNA
gtttactcccagcatcactt

SEQ ID NO: 11670 - RNA, 20 nt, synthetic construct
  source 1..20: mol_type = other RNA
agtttactcccagcatcact

SEQ ID NO: 11671 - RNA, 20 nt, synthetic construct
  source 1..20: mol_type = other RNA
tgagagtcacaaacatgttt

SEQ ID NO: 11672 - RNA, 20 nt, synthetic construct
  source 1..20: mol_type = other RNA
gttttggcaatataaccaga

SEQ ID NO: 11673 - RNA, 20 nt, synthetic construct
  source 1..20: mol_type = other RNA
ttttggcaatataaccagat

SEQ ID NO: 11674 - RNA, 20 nt, synthetic construct
  source 1..20: mol_type = other RNA
gcaatataaccagatgggac

SEQ ID NO: 11675 - RNA, 20 nt, synthetic construct
  source 1..20: mol_type = other RNA
ttaatttctccagtcccatc

SEQ ID NO: 11676 - RNA, 20 nt, synthetic construct
  source 1..20: mol_type = other RNA
agcttagtcttgctttttta

SEQ ID NO: 11677 - RNA, 20 nt, synthetic construct
  source 1..20: mol_type = other RNA
aaaagcaagactaagctgcg

SEQ ID NO: 11678 - RNA, 20 nt, synthetic construct
  source 1..20: mol_type = other RNA
aaagcaagactaagctgcgt

SEQ ID NO: 11679 - RNA, 20 nt, synthetic construct
  source 1..20: mol_type = other RNA
gcaagactaagctgcgtggg

SEQ ID NO: 11680 - RNA, 20 nt, synthetic construct
  source 1..20: mol_type = other RNA
gctgcgtgggaggccaaacg

SEQ ID NO: 11681 - RNA, 20 nt, synthetic construct
  source 1..20: mol_type = other RNA
ctgcgtgggaggccaaacga

SEQ ID NO: 11682 - RNA, 20 nt, synthetic construct
  source 1..20: mol_type = other RNA
tgcgtgggaggccaaacgag

SEQ ID NO: 11683 - RNA, 20 nt, synthetic construct
  source 1..20: mol_type = other RNA
gcgtgggaggccaaacgagg

SEQ ID NO: 11684 - RNA, 20 nt, synthetic construct
  source 1..20: mol_type = other RNA
cgtgggaggccaaacgaggg

SEQ ID NO: 11685 - RNA, 20 nt, synthetic construct
  source 1..20: mol_type = other RNA
gccaaacgaggggggtcctt

SEQ ID NO: 11686 - RNA, 20 nt, synthetic construct
  source 1..20: mol_type = other RNA
ccaaacgaggggggtccttt

SEQ ID NO: 11687 - RNA, 20 nt, synthetic construct
  source 1..20: mol_type = other RNA
cccaaaggacccccctcgtt

SEQ ID NO: 11688 - RNA, 20 nt, synthetic construct
  source 1..20: mol_type = other RNA
tcatggtagaaacagcccaa

SEQ ID NO: 11689 - RNA, 20 nt, synthetic construct
  source 1..20: mol_type = other RNA
ggtaatggcgatttttgtca

SEQ ID NO: 11690 - RNA, 20 nt, synthetic construct
  source 1..20: mol_type = other RNA
gtgtgagaggtgtggggtaa

SEQ ID NO: 11691 - RNA, 20 nt, synthetic construct
  source 1..20: mol_type = other RNA
ttggcggtgtgagaggtgtg

SEQ ID NO: 11692 - RNA, 20 nt, synthetic construct
  source 1..20: mol_type = other RNA
gttggcggtgtgagaggtgt

SEQ ID NO: 11693 - RNA, 20 nt, synthetic construct
  source 1..20: mol_type = other RNA
cgttggcggtgtgagaggtg

SEQ ID NO: 11694 - RNA, 20 nt, synthetic construct
  source 1..20: mol_type = other RNA
cggaacgttggcggtgtgag

SEQ ID NO: 11695 - RNA, 20 nt, synthetic construct
  source 1..20: mol_type = other RNA
gaacgttggcggaacgttgg

SEQ ID NO: 11696 - RNA, 20 nt, synthetic construct
  source 1..20: mol_type = other RNA
gcggaacgttggcggaacgt

SEQ ID NO: 11697 - RNA, 20 nt, synthetic construct
  source 1..20: mol_type = other RNA
ggacgttggcggaacgttgg

SEQ ID NO: 11698 - RNA, 20 nt, synthetic construct
  source 1..20: mol_type = other RNA
gtgggacgttggcggaacgt

SEQ ID NO: 11699 - RNA, 20 nt, synthetic construct
  source 1..20: mol_type = other RNA
tgagggtggtgggacgttgg

SEQ ID NO: 11700 - RNA, 20 nt, synthetic construct
  source 1..20: mol_type = other RNA
tcatgagggtggtgggacgt

SEQ ID NO: 11701 - RNA, 20 nt, synthetic construct
  source 1..20: mol_type = other RNA
acggatatcatgagggtggt

SEQ ID NO: 11702 - RNA, 20 nt, synthetic construct
  source 1..20: mol_type = other RNA
gacggatatcatgagggtgg

SEQ ID NO: 11703 - RNA, 20 nt, synthetic construct
  source 1..20: mol_type = other RNA
gcggacggatatcatgaggg

SEQ ID NO: 11704 - RNA, 20 nt, synthetic construct
  source 1..20: mol_type = other RNA
accgcggacggatatcatga

SEQ ID NO: 11705 - RNA, 20 nt, synthetic construct
  source 1..20: mol_type = other RNA
taccgcggacggatatcatg

SEQ ID NO: 11706 - RNA, 20 nt, synthetic construct
  source 1..20: mol_type = other RNA
ccgcggtactgctccagcga

SEQ ID NO: 11707 - RNA, 20 nt, synthetic construct
  source 1..20: mol_type = other RNA
cgctggagcagtaccgcgga

SEQ ID NO: 11708 - RNA, 20 nt, synthetic construct
  source 1..20: mol_type = other RNA
ccttcgctggagcagtaccg

SEQ ID NO: 11709 - RNA, 20 nt, synthetic construct
  source 1..20: mol_type = other RNA
ccagcgaaggtacccttgcc

SEQ ID NO: 11710 - RNA, 20 nt, synthetic construct
  source 1..20: mol_type = other RNA
cagcgaaggtacccttgcct

SEQ ID NO: 11711 - RNA, 20 nt, synthetic construct
  source 1..20: mol_type = other RNA
ccaggcaagggtaccttcgc

SEQ ID NO: 11712 - RNA, 20 nt, synthetic construct
  source 1..20: mol_type = other RNA
gtacccttgcctgggccatg

SEQ ID NO: 11713 - RNA, 20 nt, synthetic construct
  source 1..20: mol_type = other RNA
gcgcctcatggcccaggcaa

SEQ ID NO: 11714 - RNA, 20 nt, synthetic construct
  source 1..20: mol_type = other RNA
tgcgcctcatggcccaggca

SEQ ID NO: 11715 - RNA, 20 nt, synthetic construct
  source 1..20: mol_type = other RNA
acggttgcgcctcatggccc

SEQ ID NO: 11716 - RNA, 20 nt, synthetic construct
  source 1..20: mol_type = other RNA
tgagggacggttgcgcctca

SEQ ID NO: 11717 - RNA, 20 nt, synthetic construct
  source 1..20: mol_type = other RNA
gcgcaaccgtccctcacagc

SEQ ID NO: 11718 - RNA, 20 nt, synthetic construct
  source 1..20: mol_type = other RNA
cgcaaccgtccctcacagct

SEQ ID NO: 11719 - RNA, 20 nt, synthetic construct
  source 1..20: mol_type = other RNA
gcaaccgtccctcacagctg

SEQ ID NO: 11720 - RNA, 20 nt, synthetic construct
  source 1..20: mol_type = other RNA
accgtccctcacagctgggg

SEQ ID NO: 11721 - RNA, 20 nt, synthetic construct
  source 1..20: mol_type = other RNA
gccaccccagctgtgaggga

SEQ ID NO: 11722 - RNA, 20 nt, synthetic construct
  source 1..20: mol_type = other RNA
agaagccaccccagctgtga

SEQ ID NO: 11723 - RNA, 20 nt, synthetic construct
  source 1..20: mol_type = other RNA
gagaagccaccccagctgtg

SEQ ID NO: 11724 - RNA, 20 nt, synthetic construct
  source 1..20: mol_type = other RNA
gcttctccaggttcgcaccg

SEQ ID NO: 11725 - RNA, 20 nt, synthetic construct
  source 1..20: mol_type = other RNA
cttctccaggttcgcaccga

SEQ ID NO: 11726 - RNA, 20 nt, synthetic construct
  source 1..20: mol_type = other RNA
ttctccaggttcgcaccgag

SEQ ID NO: 11727 - RNA, 20 nt, synthetic construct
  source 1..20: mol_type = other RNA
ggttcgcaccgaggggaagt

SEQ ID NO: 11728 - RNA, 20 nt, synthetic construct
  source 1..20: mol_type = other RNA
gttcgcaccgaggggaagtt

SEQ ID NO: 11729 - RNA, 20 nt, synthetic construct
  source 1..20: mol_type = other RNA
acttcccctcggtgcgaacc

SEQ ID NO: 11730 - RNA, 20 nt, synthetic construct
  source 1..20: mol_type = other RNA
ccgaggggaagttggggtac

SEQ ID NO: 11731 - RNA, 20 nt, synthetic construct
  source 1..20: mol_type = other RNA
ccggtaccccaacttcccct

SEQ ID NO: 11732 - RNA, 20 nt, synthetic construct
  source 1..20: mol_type = other RNA
tgggtgctggcggcggaaac

SEQ ID NO: 11733 - RNA, 20 nt, synthetic construct
  source 1..20: mol_type = other RNA
tccgccgccagcacccaaga

SEQ ID NO: 11734 - RNA, 20 nt, synthetic construct
  source 1..20: mol_type = other RNA
gccgccagcacccaagatgg

SEQ ID NO: 11735 - RNA, 20 nt, synthetic construct
  source 1..20: mol_type = other RNA
gccatcttgggtgctggcgg

SEQ ID NO: 11736 - RNA, 20 nt, synthetic construct
  source 1..20: mol_type = other RNA
gccgccatcttgggtgctgg

SEQ ID NO: 11737 - RNA, 20 nt, synthetic construct
  source 1..20: mol_type = other RNA
cgtgccgccatcttgggtgc

SEQ ID NO: 11738 - RNA, 20 nt, synthetic construct
  source 1..20: mol_type = other RNA
gacgctcgtgccgccatctt

SEQ ID NO: 11739 - RNA, 20 nt, synthetic construct
  source 1..20: mol_type = other RNA
cgacgctcgtgccgccatct

SEQ ID NO: 11740 - RNA, 20 nt, synthetic construct
  source 1..20: mol_type = other RNA
cacgaagcatgtggttcttg

SEQ ID NO: 11741 - RNA, 20 nt, synthetic construct
  source 1..20: mol_type = other RNA
gaggcgggacacgaagcatg

SEQ ID NO: 11742 - RNA, 20 nt, synthetic construct
  source 1..20: mol_type = other RNA
gtgtcccgcctcagcattct

SEQ ID NO: 11743 - RNA, 20 nt, synthetic construct
  source 1..20: mol_type = other RNA
tgtcccgcctcagcattctc

SEQ ID NO: 11744 - RNA, 20 nt, synthetic construct
  source 1..20: mol_type = other RNA
agacccgagaatgctgaggc

SEQ ID NO: 11745 - RNA, 20 nt, synthetic construct
  source 1..20: mol_type = other RNA
gagacccgagaatgctgagg

SEQ ID NO: 11746 - RNA, 20 nt, synthetic construct
  source 1..20: mol_type = other RNA
agtgagacccgagaatgctg

SEQ ID NO: 11747 - RNA, 20 nt, synthetic construct
  source 1..20: mol_type = other RNA
tagacttttgcaagtcactg

SEQ ID NO: 11748 - RNA, 20 nt, synthetic construct
  source 1..20: mol_type = other RNA
agacttttgcaagtcactgt

SEQ ID NO: 11749 - RNA, 20 nt, synthetic construct
  source 1..20: mol_type = other RNA
agtcactgtgggaaccctca

SEQ ID NO: 11750 - RNA, 20 nt, synthetic construct
  source 1..20: mol_type = other RNA
ctgtgggaaccctcaaggcg

SEQ ID NO: 11751 - RNA, 20 nt, synthetic construct
  source 1..20: mol_type = other RNA
tgtgggaaccctcaaggcga

SEQ ID NO: 11752 - RNA, 20 nt, synthetic construct
  source 1..20: mol_type = other RNA
gcggaacaccctcgccttga

SEQ ID NO: 11753 - RNA, 20 nt, synthetic construct
  source 1..20: mol_type = other RNA
tgcggaacaccctcgccttg

SEQ ID NO: 11754 - RNA, 20 nt, synthetic construct
  source 1..20: mol_type = other RNA
ggcgagggtgttccgcactc

SEQ ID NO: 11755 - RNA, 20 nt, synthetic construct
  source 1..20: mol_type = other RNA
gagggtgttccgcactctgg

SEQ ID NO: 11756 - RNA, 20 nt, synthetic construct
  source 1..20: mol_type = other RNA
ggtgtatcgccgccagagtg

SEQ ID NO: 11757 - RNA, 20 nt, synthetic construct
  source 1..20: mol_type = other RNA
accttcctattccctgacct

SEQ ID NO: 11758 - RNA, 20 nt, synthetic construct
  source 1..20: mol_type = other RNA
gcctaggtcagggaatagga

SEQ ID NO: 11759 - RNA, 20 nt, synthetic construct
  source 1..20: mol_type = other RNA
gaaggcctaggtcagggaat

SEQ ID NO: 11760 - RNA, 20 nt, synthetic construct
  source 1..20: mol_type = other RNA
gggaatgaaggcctaggtca

SEQ ID NO: 11761 - RNA, 20 nt, synthetic construct
  source 1..20: mol_type = other RNA
ggggaatgaaggcctaggtc

SEQ ID NO: 11762 - RNA, 20 nt, synthetic construct
  source 1..20: mol_type = other RNA
tggcgggggaatgaaggcct

SEQ ID NO: 11763 - RNA, 20 nt, synthetic construct
  source 1..20: mol_type = other RNA
tttctgtggcgggggaatga

SEQ ID NO: 11764 - RNA, 20 nt, synthetic construct
  source 1..20: mol_type = other RNA
tcccccgccacagaaagcgc

SEQ ID NO: 11765 - RNA, 20 nt, synthetic construct
  source 1..20: mol_type = other RNA
tccagcgctttctgtggcgg

SEQ ID NO: 11766 - RNA, 20 nt, synthetic construct
  source 1..20: mol_type = other RNA
ttccagcgctttctgtggcg

SEQ ID NO: 11767 - RNA, 20 nt, synthetic construct
  source 1..20: mol_type = other RNA
cttccagcgctttctgtggc

SEQ ID NO: 11768 - RNA, 20 nt, synthetic construct
  source 1..20: mol_type = other RNA
gcttccagcgctttctgtgg

SEQ ID NO: 11769 - RNA, 20 nt, synthetic construct
  source 1..20: mol_type = other RNA
ggcgcttccagcgctttctg

SEQ ID NO: 11770 - RNA, 20 nt, synthetic construct
  source 1..20: mol_type = other RNA
agcgctggaagcgcccaacc

SEQ ID NO: 11771 - RNA, 20 nt, synthetic construct
  source 1..20: mol_type = other RNA
ttgggtgaagtatccaggtt

SEQ ID NO: 11772 - RNA, 20 nt, synthetic construct
  source 1..20: mol_type = other RNA
gttgggtgaagtatccaggt

SEQ ID NO: 11773 - RNA, 20 nt, synthetic construct
  source 1..20: mol_type = other RNA
gggcgttgggtgaagtatcc

SEQ ID NO: 11774 - RNA, 20 nt, synthetic construct
  source 1..20: mol_type = other RNA
tgttagtgggcttgggcgtt

SEQ ID NO: 11775 - RNA, 20 nt, synthetic construct
  source 1..20: mol_type = other RNA
atgttagtgggcttgggcgt

SEQ ID NO: 11776 - RNA, 20 nt, synthetic construct
  source 1..20: mol_type = other RNA
cgggcgatgttagtgggctt

SEQ ID NO: 11777 - RNA, 20 nt, synthetic construct
  source 1..20: mol_type = other RNA
gcgggcgatgttagtgggct

SEQ ID NO: 11778 - RNA, 20 nt, synthetic construct
  source 1..20: mol_type = other RNA
actaacatcgcccgccgcga

SEQ ID NO: 11779 - RNA, 20 nt, synthetic construct
  source 1..20: mol_type = other RNA
tcgcggcgggcgatgttagt

SEQ ID NO: 11780 - RNA, 20 nt, synthetic construct
  source 1..20: mol_type = other RNA
ttcgcggcgggcgatgttag

SEQ ID NO: 11781 - RNA, 20 nt, synthetic construct
  source 1..20: mol_type = other RNA
catcgcccgccgcgaaggcg

SEQ ID NO: 11782 - RNA, 20 nt, synthetic construct
  source 1..20: mol_type = other RNA
ccgccgcgaaggcgcggccg

SEQ ID NO: 11783 - RNA, 20 nt, synthetic construct
  source 1..20: mol_type = other RNA
cgccgcgaaggcgcggccga

SEQ ID NO: 11784 - RNA, 20 nt, synthetic construct
  source 1..20: mol_type = other RNA
gccgcgaaggcgcggccgag

SEQ ID NO: 11785 - RNA, 20 nt, synthetic construct
  source 1..20: mol_type = other RNA
ctcggccgcgccttcgcggc

SEQ ID NO: 11786 - RNA, 20 nt, synthetic construct
  source 1..20: mol_type = other RNA
cctcggccgcgccttcgcgg

SEQ ID NO: 11787 - RNA, 20 nt, synthetic construct
  source 1..20: mol_type = other RNA
gcccctcggccgcgccttcg

SEQ ID NO: 11788 - RNA, 20 nt, synthetic construct
  source 1..20: mol_type = other RNA
gtctggcattctgggcccct

SEQ ID NO: 11789 - RNA, 20 nt, synthetic construct
  source 1..20: mol_type = other RNA
ggcccagaatgccagacact

SEQ ID NO: 11790 - RNA, 20 nt, synthetic construct
  source 1..20: mol_type = other RNA
gcccagaatgccagacacta

SEQ ID NO: 11791 - RNA, 20 nt, synthetic construct
  source 1..20: mol_type = other RNA
gccctagtgtctggcattct

SEQ ID NO: 11792 - RNA, 20 nt, synthetic construct
  source 1..20: mol_type = other RNA
ggccctagtgtctggcattc

SEQ ID NO: 11793 - RNA, 20 nt, synthetic construct
  source 1..20: mol_type = other RNA
agggcgaaggccctagtgtc

SEQ ID NO: 11794 - RNA, 20 nt, synthetic construct
  source 1..20: mol_type = other RNA
agggccttcgccctcctcat

SEQ ID NO: 11795 - RNA, 20 nt, synthetic construct
  source 1..20: mol_type = other RNA
gccttcgccctcctcattgg

SEQ ID NO: 11796 - RNA, 20 nt, synthetic construct
  source 1..20: mol_type = other RNA
ccttcgccctcctcattggt

SEQ ID NO: 11797 - RNA, 20 nt, synthetic construct
  source 1..20: mol_type = other RNA
cccaccaatgaggagggcga

SEQ ID NO: 11798 - RNA, 20 nt, synthetic construct
  source 1..20: mol_type = other RNA
tatggacccaccaatgagga

SEQ ID NO: 11799 - RNA, 20 nt, synthetic construct
  source 1..20: mol_type = other RNA
tcattggtgggtccataccg

SEQ ID NO: 11800 - RNA, 20 nt, synthetic construct
  source 1..20: mol_type = other RNA
cattggtgggtccataccgc

SEQ ID NO: 11801 - RNA, 20 nt, synthetic construct
  source 1..20: mol_type = other RNA
attggtgggtccataccgcg

SEQ ID NO: 11802 - RNA, 20 nt, synthetic construct
  source 1..20: mol_type = other RNA
gcggtatggacccaccaatg

SEQ ID NO: 11803 - RNA, 20 nt, synthetic construct
  source 1..20: mol_type = other RNA
ggtgggtccataccgcgggg

SEQ ID NO: 11804 - RNA, 20 nt, synthetic construct
  source 1..20: mol_type = other RNA
gtgggtccataccgcggggc

SEQ ID NO: 11805 - RNA, 20 nt, synthetic construct
  source 1..20: mol_type = other RNA
ccataccgcggggcgggcct

SEQ ID NO: 11806 - RNA, 20 nt, synthetic construct
  source 1..20: mol_type = other RNA
cctaggcccgccccgcggta

SEQ ID NO: 11807 - RNA, 20 nt, synthetic construct
  source 1..20: mol_type = other RNA
gagtacctaggcccgccccg

SEQ ID NO: 11808 - RNA, 20 nt, synthetic construct
  source 1..20: mol_type = other RNA
ggcgggcctaggtactcatt

SEQ ID NO: 11809 - RNA, 20 nt, synthetic construct
  source 1..20: mol_type = other RNA
ggcctaggtactcattgggc

SEQ ID NO: 11810 - RNA, 20 nt, synthetic construct
  source 1..20: mol_type = other RNA
gcctaggtactcattgggcc

SEQ ID NO: 11811 - RNA, 20 nt, synthetic construct
  source 1..20: mol_type = other RNA
tcccggcccaatgagtacct

SEQ ID NO: 11812 - RNA, 20 nt, synthetic construct
  source 1..20: mol_type = other RNA
gccgggaattatgtcagtct

SEQ ID NO: 11813 - RNA, 20 nt, synthetic construct
  source 1..20: mol_type = other RNA
ccgggaattatgtcagtctt

SEQ ID NO: 11814 - RNA, 20 nt, synthetic construct
  source 1..20: mol_type = other RNA
cccaagactgacataattcc

SEQ ID NO: 11815 - RNA, 20 nt, synthetic construct
  source 1..20: mol_type = other RNA
tatgtcagtcttgggaaatc

SEQ ID NO: 11816 - RNA, 20 nt, synthetic construct
  source 1..20: mol_type = other RNA
cagtcttgggaaatcaggtc

SEQ ID NO: 11817 - RNA, 20 nt, synthetic construct
  source 1..20: mol_type = other RNA
agtcttgggaaatcaggtcc

SEQ ID NO: 11818 - RNA, 20 nt, synthetic construct
  source 1..20: mol_type = other RNA
gtcttgggaaatcaggtccg

SEQ ID NO: 11819 - RNA, 20 nt, synthetic construct
  source 1..20: mol_type = other RNA
ggaaatcaggtccggggatg

SEQ ID NO: 11820 - RNA, 20 nt, synthetic construct
  source 1..20: mol_type = other RNA
aatcaggtccggggatgagg

SEQ ID NO: 11821 - RNA, 20 nt, synthetic construct
  source 1..20: mol_type = other RNA
tgagtgtacctcctcatccc

SEQ ID NO: 11822 - RNA, 20 nt, synthetic construct
  source 1..20: mol_type = other RNA
gaggaggtacactcagccat

SEQ ID NO: 11823 - RNA, 20 nt, synthetic construct
  source 1..20: mol_type = other RNA
aggaggtacactcagccatt

SEQ ID NO: 11824 - RNA, 20 nt, synthetic construct
  source 1..20: mol_type = other RNA
tggcagcagagagggcccaa

SEQ ID NO: 11825 - RNA, 20 nt, synthetic construct
  source 1..20: mol_type = other RNA
ccctctctgctgccaatcag

SEQ ID NO: 11826 - RNA, 20 nt, synthetic construct
  source 1..20: mol_type = other RNA
cctctctgctgccaatcaga

SEQ ID NO: 11827 - RNA, 20 nt, synthetic construct
  source 1..20: mol_type = other RNA
cctctgattggcagcagaga

SEQ ID NO: 11828 - RNA, 20 nt, synthetic construct
  source 1..20: mol_type = other RNA
ccctctgattggcagcagag

SEQ ID NO: 11829 - RNA, 20 nt, synthetic construct
  source 1..20: mol_type = other RNA
atcagagggacatccgtcga

SEQ ID NO: 11830 - RNA, 20 nt, synthetic construct
  source 1..20: mol_type = other RNA
tcgacggatgtccctctgat

SEQ ID NO: 11831 - RNA, 20 nt, synthetic construct
  source 1..20: mol_type = other RNA
gggacatccgtcgacggccc

SEQ ID NO: 11832 - RNA, 20 nt, synthetic construct
  source 1..20: mol_type = other RNA
tccgtcgacggccccggcct

SEQ ID NO: 11833 - RNA, 20 nt, synthetic construct
  source 1..20: mol_type = other RNA
gccgaggccggggccgtcga

SEQ ID NO: 11834 - RNA, 20 nt, synthetic construct
  source 1..20: mol_type = other RNA
cccggcctcggctcgttgat

SEQ ID NO: 11835 - RNA, 20 nt, synthetic construct
  source 1..20: mol_type = other RNA
caatcaacgagccgaggccg

SEQ ID NO: 11836 - RNA, 20 nt, synthetic construct
  source 1..20: mol_type = other RNA
ccaatcaacgagccgaggcc

SEQ ID NO: 11837 - RNA, 20 nt, synthetic construct
  source 1..20: mol_type = other RNA
tccaatcaacgagccgaggc

SEQ ID NO: 11838 - RNA, 20 nt, synthetic construct
  source 1..20: mol_type = other RNA
tttctccaatcaacgagccg

SEQ ID NO: 11839 - RNA, 20 nt, synthetic construct
  source 1..20: mol_type = other RNA
tgattggagaaactgttcct

SEQ ID NO: 11840 - RNA, 20 nt, synthetic construct
  source 1..20: mol_type = other RNA
gattggagaaactgttccta

SEQ ID NO: 11841 - RNA, 20 nt, synthetic construct
  source 1..20: mol_type = other RNA
aactgttcctagggtgtttg

SEQ ID NO: 11842 - RNA, 20 nt, synthetic construct
  source 1..20: mol_type = other RNA
tgttcctagggtgtttgcgg

SEQ ID NO: 11843 - RNA, 20 nt, synthetic construct
  source 1..20: mol_type = other RNA
gttcctagggtgtttgcggc

SEQ ID NO: 11844 - RNA, 20 nt, synthetic construct
  source 1..20: mol_type = other RNA
cctagggtgtttgcggcggg

SEQ ID NO: 11845 - RNA, 20 nt, synthetic construct
  source 1..20: mol_type = other RNA
ctagggtgtttgcggcgggc

SEQ ID NO: 11846 - RNA, 20 nt, synthetic construct
  source 1..20: mol_type = other RNA
ccgcccgccgcaaacaccct

SEQ ID NO: 11847 - RNA, 20 nt, synthetic construct
  source 1..20: mol_type = other RNA
ggcgggcgggtttccgagtg

SEQ ID NO: 11848 - RNA, 20 nt, synthetic construct
  source 1..20: mol_type = other RNA
gggtttccgagtgcggtagc

SEQ ID NO: 11849 - RNA, 20 nt, synthetic construct
  source 1..20: mol_type = other RNA
tttccgagtgcggtagcagg

SEQ ID NO: 11850 - RNA, 20 nt, synthetic construct
  source 1..20: mol_type = other RNA
ttccgagtgcggtagcagga

SEQ ID NO: 11851 - RNA, 20 nt, synthetic construct
  source 1..20: mol_type = other RNA
tccgagtgcggtagcaggag

SEQ ID NO: 11852 - RNA, 20 nt, synthetic construct
  source 1..20: mol_type = other RNA
ccgagtgcggtagcaggagg

SEQ ID NO: 11853 - RNA, 20 nt, synthetic construct
  source 1..20: mol_type = other RNA
agtgcggtagcaggaggggg

SEQ ID NO: 11854 - RNA, 20 nt, synthetic construct
  source 1..20: mol_type = other RNA
gtgcggtagcaggagggggc

SEQ ID NO: 11855 - RNA, 20 nt, synthetic construct
  source 1..20: mol_type = other RNA
ccccctcctgctaccgcact

SEQ ID NO: 11856 - RNA, 20 nt, synthetic construct
  source 1..20: mol_type = other RNA
ggtagcaggagggggcgggg

SEQ ID NO: 11857 - RNA, 20 nt, synthetic construct
  source 1..20: mol_type = other RNA
ggagggggcggggaggtaag

SEQ ID NO: 11858 - RNA, 20 nt, synthetic construct
  source 1..20: mol_type = other RNA
gggggcggggaggtaagcgg

SEQ ID NO: 11859 - RNA, 20 nt, synthetic construct
  source 1..20: mol_type = other RNA
aagcggaggctccgagctct

SEQ ID NO: 11860 - RNA, 20 nt, synthetic construct
  source 1..20: mol_type = other RNA
ggaggctccgagctctaggc

SEQ ID NO: 11861 - RNA, 20 nt, synthetic construct
  source 1..20: mol_type = other RNA
gctccgagctctaggccggc

SEQ ID NO: 11862 - RNA, 20 nt, synthetic construct
  source 1..20: mol_type = other RNA
ccgagctctaggccggccgg

SEQ ID NO: 11863 - RNA, 20 nt, synthetic construct
  source 1..20: mol_type = other RNA
agctctaggccggccggcgg

SEQ ID NO: 11864 - RNA, 20 nt, synthetic construct
  source 1..20: mol_type = other RNA
ccgccggccggcctagagct

SEQ ID NO: 11865 - RNA, 20 nt, synthetic construct
  source 1..20: mol_type = other RNA
tctaggccggccggcggtgg

SEQ ID NO: 11866 - RNA, 20 nt, synthetic construct
  source 1..20: mol_type = other RNA
aggccggccggcggtggcgg

SEQ ID NO: 11867 - RNA, 20 nt, synthetic construct
  source 1..20: mol_type = other RNA
ggccggcggtggcggcggcg

SEQ ID NO: 11868 - RNA, 20 nt, synthetic construct
  source 1..20: mol_type = other RNA
tcgccgccgccaccgccggc

SEQ ID NO: 11869 - RNA, 20 nt, synthetic construct
  source 1..20: mol_type = other RNA
ggcggtggcggcggcgaggc

SEQ ID NO: 11870 - RNA, 20 nt, synthetic construct
  source 1..20: mol_type = other RNA
gcggtggcggcggcgaggcc

SEQ ID NO: 11871 - RNA, 20 nt, synthetic construct
  source 1..20: mol_type = other RNA
ggcctcgccgccgccaccgc

SEQ ID NO: 11872 - RNA, 20 nt, synthetic construct
  source 1..20: mol_type = other RNA
gcggcggcgaggccgggact

SEQ ID NO: 11873 - RNA, 20 nt, synthetic construct
  source 1..20: mol_type = other RNA
cggcggcgaggccgggactc

SEQ ID NO: 11874 - RNA, 20 nt, synthetic construct
  source 1..20: mol_type = other RNA
cgaggccgggactcgggctt

SEQ ID NO: 11875 - RNA, 20 nt, synthetic construct
  source 1..20: mol_type = other RNA
gaggccgggactcgggctta

SEQ ID NO: 11876 - RNA, 20 nt, synthetic construct
  source 1..20: mol_type = other RNA
caggccctaagcccgagtcc

SEQ ID NO: 11877 - RNA, 20 nt, synthetic construct
  source 1..20: mol_type = other RNA
ctcgggcttagggcctgctg

SEQ ID NO: 11878 - RNA, 20 nt, synthetic construct
  source 1..20: mol_type = other RNA
gggcttagggcctgctgtgg

SEQ ID NO: 11879 - RNA, 20 nt, synthetic construct
  source 1..20: mol_type = other RNA
agggcctgctgtggaggcag

SEQ ID NO: 11880 - RNA, 20 nt, synthetic construct
  source 1..20: mol_type = other RNA
gcctgctgtggaggcagcgg

SEQ ID NO: 11881 - RNA, 20 nt, synthetic construct
  source 1..20: mol_type = other RNA
tccgccgctgcctccacagc

SEQ ID NO: 11882 - RNA, 20 nt, synthetic construct
  source 1..20: mol_type = other RNA
gcggacgccgagctaagcag

SEQ ID NO: 11883 - RNA, 20 nt, synthetic construct
  source 1..20: mol_type = other RNA
cggacgccgagctaagcagt

SEQ ID NO: 11884 - RNA, 20 nt, synthetic construct
  source 1..20: mol_type = other RNA
ccgagctaagcagtgggtat

SEQ ID NO: 11885 - RNA, 20 nt, synthetic construct
  source 1..20: mol_type = other RNA
cgagctaagcagtgggtatc

SEQ ID NO: 11886 - RNA, 20 nt, synthetic construct
  source 1..20: mol_type = other RNA
ccgatacccactgcttagct

SEQ ID NO: 11887 - RNA, 20 nt, synthetic construct
  source 1..20: mol_type = other RNA
gggcacattcctttcccaga

SEQ ID NO: 11888 - RNA, 20 nt, synthetic construct
  source 1..20: mol_type = other RNA
ggcacattcctttcccagaa

SEQ ID NO: 11889 - RNA, 20 nt, synthetic construct
  source 1..20: mol_type = other RNA
acattcctttcccagaaggg

SEQ ID NO: 11890 - RNA, 20 nt, synthetic construct
  source 1..20: mol_type = other RNA
cattcctttcccagaaggga

SEQ ID NO: 11891 - RNA, 20 nt, synthetic construct
  source 1..20: mol_type = other RNA
gcaaccctcccttctgggaa

SEQ ID NO: 11892 - RNA, 20 nt, synthetic construct
  source 1..20: mol_type = other RNA
aagggagggttgcagcgccg

SEQ ID NO: 11893 - RNA, 20 nt, synthetic construct
  source 1..20: mol_type = other RNA
agggagggttgcagcgccgc

SEQ ID NO: 11894 - RNA, 20 nt, synthetic construct
  source 1..20: mol_type = other RNA
gggagggttgcagcgccgcg

SEQ ID NO: 11895 - RNA, 20 nt, synthetic construct
  source 1..20: mol_type = other RNA
gttgcagcgccgcggggccg

SEQ ID NO: 11896 - RNA, 20 nt, synthetic construct
  source 1..20: mol_type = other RNA
cgccgcggggccgaggctta

SEQ ID NO: 11897 - RNA, 20 nt, synthetic construct
  source 1..20: mol_type = other RNA
gccgcggggccgaggcttat

SEQ ID NO: 11898 - RNA, 20 nt, synthetic construct
  source 1..20: mol_type = other RNA
ccgcggggccgaggcttatg

SEQ ID NO: 11899 - RNA, 20 nt, synthetic construct
  source 1..20: mol_type = other RNA
ccccataagcctcggccccg

SEQ ID NO: 11900 - RNA, 20 nt, synthetic construct
  source 1..20: mol_type = other RNA
ggccgaggcttatggggcga

SEQ ID NO: 11901 - RNA, 20 nt, synthetic construct
  source 1..20: mol_type = other RNA
gccgaggcttatggggcgac

SEQ ID NO: 11902 - RNA, 20 nt, synthetic construct
  source 1..20: mol_type = other RNA
aggcttatggggcgacggga

SEQ ID NO: 11903 - RNA, 20 nt, synthetic construct
  source 1..20: mol_type = other RNA
tcccgtcgccccataagcct

SEQ ID NO: 11904 - RNA, 20 nt, synthetic construct
  source 1..20: mol_type = other RNA
ggggcgacgggatggtgctg

SEQ ID NO: 11905 - RNA, 20 nt, synthetic construct
  source 1..20: mol_type = other RNA
acgggatggtgctgaggtgc

SEQ ID NO: 11906 - RNA, 20 nt, synthetic construct
  source 1..20: mol_type = other RNA
ggatggtgctgaggtgcagg

SEQ ID NO: 11907 - RNA, 20 nt, synthetic construct
  source 1..20: mol_type = other RNA
tggtgctgaggtgcaggagg

SEQ ID NO: 11908 - RNA, 20 nt, synthetic construct
  source 1..20: mol_type = other RNA
ggtgctgaggtgcaggaggc

SEQ ID NO: 11909 - RNA, 20 nt, synthetic construct
  source 1..20: mol_type = other RNA
gtgctgaggtgcaggaggcg

SEQ ID NO: 11910 - RNA, 20 nt, synthetic construct
  source 1..20: mol_type = other RNA
tgctgaggtgcaggaggcgg

SEQ ID NO: 11911 - RNA, 20 nt, synthetic construct
  source 1..20: mol_type = other RNA
tgcaggaggcgggggccgag

SEQ ID NO: 11912 - RNA, 20 nt, synthetic construct
  source 1..20: mol_type = other RNA
gcaggaggcgggggccgagc

SEQ ID NO: 11913 - RNA, 20 nt, synthetic construct
  source 1..20: mol_type = other RNA
caggaggcgggggccgagcg

SEQ ID NO: 11914 - RNA, 20 nt, synthetic construct
  source 1..20: mol_type = other RNA
gcggggttcccgccagagcc

SEQ ID NO: 11915 - RNA, 20 nt, synthetic construct
  source 1..20: mol_type = other RNA
gctctggcgggaaccccgct

SEQ ID NO: 11916 - RNA, 20 nt, synthetic construct
  source 1..20: mol_type = other RNA
ttcccgccagagcccggccc

SEQ ID NO: 11917 - RNA, 20 nt, synthetic construct
  source 1..20: mol_type = other RNA
tcccgccagagcccggccct

SEQ ID NO: 11918 - RNA, 20 nt, synthetic construct
  source 1..20: mol_type = other RNA
gcccagggccgggctctggc

SEQ ID NO: 11919 - RNA, 20 nt, synthetic construct
  source 1..20: mol_type = other RNA
ggcccagggccgggctctgg

SEQ ID NO: 11920 - RNA, 20 nt, synthetic construct
  source 1..20: mol_type = other RNA
agcccggccctgggcctgac

SEQ ID NO: 11921 - RNA, 20 nt, synthetic construct
  source 1..20: mol_type = other RNA
gcccggccctgggcctgaca

SEQ ID NO: 11922 - RNA, 20 nt, synthetic construct
  source 1..20: mol_type = other RNA
cggccctgggcctgacaggg

SEQ ID NO: 11923 - RNA, 20 nt, synthetic construct
  source 1..20: mol_type = other RNA
ggccctgggcctgacaggga

SEQ ID NO: 11924 - RNA, 20 nt, synthetic construct
  source 1..20: mol_type = other RNA
gccctgggcctgacagggag

SEQ ID NO: 11925 - RNA, 20 nt, synthetic construct
  source 1..20: mol_type = other RNA
tccctgtcaggcccagggcc

SEQ ID NO: 11926 - RNA, 20 nt, synthetic construct
  source 1..20: mol_type = other RNA
ctccctgtcaggcccagggc

SEQ ID NO: 11927 - RNA, 20 nt, synthetic construct
  source 1..20: mol_type = other RNA
gcccctccctgtcaggccca

SEQ ID NO: 11928 - RNA, 20 nt, synthetic construct
  source 1..20: mol_type = other RNA
ggcccctccctgtcaggccc

SEQ ID NO: 11929 - RNA, 20 nt, synthetic construct
  source 1..20: mol_type = other RNA
tgacagggaggggccccgcg

SEQ ID NO: 11930 - RNA, 20 nt, synthetic construct
  source 1..20: mol_type = other RNA
gacagggaggggccccgcgc

SEQ ID NO: 11931 - RNA, 20 nt, synthetic construct
  source 1..20: mol_type = other RNA
acagggaggggccccgcgcg

SEQ ID NO: 11932 - RNA, 20 nt, synthetic construct
  source 1..20: mol_type = other RNA
gcgcggggcccctccctgtc

SEQ ID NO: 11933 - RNA, 20 nt, synthetic construct
  source 1..20: mol_type = other RNA
gggccccgcgcggggccgag

SEQ ID NO: 11934 - RNA, 20 nt, synthetic construct
  source 1..20: mol_type = other RNA
cgcggggccgagaggaaagc

SEQ ID NO: 11935 - RNA, 20 nt, synthetic construct
  source 1..20: mol_type = other RNA
ctttcctctcggccccgcgc

SEQ ID NO: 11936 - RNA, 20 nt, synthetic construct
  source 1..20: mol_type = other RNA
gctttcctctcggccccgcg

SEQ ID NO: 11937 - RNA, 20 nt, synthetic construct
  source 1..20: mol_type = other RNA
gccgagaggaaagctggctc

SEQ ID NO: 11938 - RNA, 20 nt, synthetic construct
  source 1..20: mol_type = other RNA
ccgagaggaaagctggctcc

SEQ ID NO: 11939 - RNA, 20 nt, synthetic construct
  source 1..20: mol_type = other RNA
cgagaggaaagctggctccg

SEQ ID NO: 11940 - RNA, 20 nt, synthetic construct
  source 1..20: mol_type = other RNA
gaggaaagctggctccgggg

SEQ ID NO: 11941 - RNA, 20 nt, synthetic construct
  source 1..20: mol_type = other RNA
aggaaagctggctccggggt

SEQ ID NO: 11942 - RNA, 20 nt, synthetic construct
  source 1..20: mol_type = other RNA
aagctggctccggggtggga

SEQ ID NO: 11943 - RNA, 20 nt, synthetic construct
  source 1..20: mol_type = other RNA
ggctccggggtgggatggac

SEQ ID NO: 11944 - RNA, 20 nt, synthetic construct
  source 1..20: mol_type = other RNA
gctccggggtgggatggact

SEQ ID NO: 11945 - RNA, 20 nt, synthetic construct
  source 1..20: mol_type = other RNA
cggggtgggatggactgggc

SEQ ID NO: 11946 - RNA, 20 nt, synthetic construct
  source 1..20: mol_type = other RNA
ggggtgggatggactgggca

SEQ ID NO: 11947 - RNA, 20 nt, synthetic construct
  source 1..20: mol_type = other RNA
ctgcccagtccatcccaccc

SEQ ID NO: 11948 - RNA, 20 nt, synthetic construct
  source 1..20: mol_type = other RNA
ggatggactgggcagggttg

SEQ ID NO: 11949 - RNA, 20 nt, synthetic construct
  source 1..20: mol_type = other RNA
gatggactgggcagggttga

SEQ ID NO: 11950 - RNA, 20 nt, synthetic construct
  source 1..20: mol_type = other RNA
gcagggttgagggcacgaga

SEQ ID NO: 11951 - RNA, 20 nt, synthetic construct
  source 1..20: mol_type = other RNA
gttgagggcacgagaaggcg

SEQ ID NO: 11952 - RNA, 20 nt, synthetic construct
  source 1..20: mol_type = other RNA
gcacgagaaggcgtggtgtg

SEQ ID NO: 11953 - RNA, 20 nt, synthetic construct
  source 1..20: mol_type = other RNA
agaaggcgtggtgtgaggcc

SEQ ID NO: 11954 - RNA, 20 nt, synthetic construct
  source 1..20: mol_type = other RNA
cgtggtgtgaggcctggact

SEQ ID NO: 11955 - RNA, 20 nt, synthetic construct
  source 1..20: mol_type = other RNA
gtggtgtgaggcctggactt

SEQ ID NO: 11956 - RNA, 20 nt, synthetic construct
  source 1..20: mol_type = other RNA
gtgaggcctggacttgggag

SEQ ID NO: 11957 - RNA, 20 nt, synthetic construct
  source 1..20: mol_type = other RNA
tgaggcctggacttgggagt

SEQ ID NO: 11958 - RNA, 20 nt, synthetic construct
  source 1..20: mol_type = other RNA
gaggcctggacttgggagtg

SEQ ID NO: 11959 - RNA, 20 nt, synthetic construct
  source 1..20: mol_type = other RNA
gcctggacttgggagtgggg

SEQ ID NO: 11960 - RNA, 20 nt, synthetic construct
  source 1..20: mol_type = other RNA
cctggacttgggagtggggt

SEQ ID NO: 11961 - RNA, 20 nt, synthetic construct
  source 1..20: mol_type = other RNA
ctggacttgggagtggggtg

SEQ ID NO: 11962 - RNA, 20 nt, synthetic construct
  source 1..20: mol_type = other RNA
cccaccccactcccaagtcc

SEQ ID NO: 11963 - RNA, 20 nt, synthetic construct
  source 1..20: mol_type = other RNA
tgggagtggggtggggccat

SEQ ID NO: 11964 - RNA, 20 nt, synthetic construct
  source 1..20: mol_type = other RNA
gggagtggggtggggccatc

SEQ ID NO: 11965 - RNA, 20 nt, synthetic construct
  source 1..20: mol_type = other RNA
gtggggtggggccatcggga

SEQ ID NO: 11966 - RNA, 20 nt, synthetic construct
  source 1..20: mol_type = other RNA
gggtggggccatcgggacgg

SEQ ID NO: 11967 - RNA, 20 nt, synthetic construct
  source 1..20: mol_type = other RNA
ggtggggccatcgggacgga

SEQ ID NO: 11968 - RNA, 20 nt, synthetic construct
  source 1..20: mol_type = other RNA
ggggccatcgggacggaggg

SEQ ID NO: 11969 - RNA, 20 nt, synthetic construct
  source 1..20: mol_type = other RNA
gggccatcgggacggagggc

SEQ ID NO: 11970 - RNA, 20 nt, synthetic construct
  source 1..20: mol_type = other RNA
ggccatcgggacggagggcg

SEQ ID NO: 11971 - RNA, 20 nt, synthetic construct
  source 1..20: mol_type = other RNA
catcgggacggagggcgggg

SEQ ID NO: 11972 - RNA, 20 nt, synthetic construct
  source 1..20: mol_type = other RNA
atcgggacggagggcggggt

SEQ ID NO: 11973 - RNA, 20 nt, synthetic construct
  source 1..20: mol_type = other RNA
tcgggacggagggcggggtg

SEQ ID NO: 11974 - RNA, 20 nt, synthetic construct
  source 1..20: mol_type = other RNA
caccccgccctccgtcccga

SEQ ID NO: 11975 - RNA, 20 nt, synthetic construct
  source 1..20: mol_type = other RNA
gcggggtggggtttgctgta

SEQ ID NO: 11976 - RNA, 20 nt, synthetic construct
  source 1..20: mol_type = other RNA
cggggtggggtttgctgtaa

SEQ ID NO: 11977 - RNA, 20 nt, synthetic construct
  source 1..20: mol_type = other RNA
ggtggggtttgctgtaaggg

SEQ ID NO: 11978 - RNA, 20 nt, synthetic construct
  source 1..20: mol_type = other RNA
gtggggtttgctgtaagggt

SEQ ID NO: 11979 - RNA, 20 nt, synthetic construct
  source 1..20: mol_type = other RNA
tttgctgtaagggtgggtca

SEQ ID NO: 11980 - RNA, 20 nt, synthetic construct
  source 1..20: mol_type = other RNA
tgtaagggtgggtcaaggcc

SEQ ID NO: 11981 - RNA, 20 nt, synthetic construct
  source 1..20: mol_type = other RNA
gtaagggtgggtcaaggcca

SEQ ID NO: 11982 - RNA, 20 nt, synthetic construct
  source 1..20: mol_type = other RNA
gggaagtagcacttgttcgc

SEQ ID NO: 11983 - RNA, 20 nt, synthetic construct
  source 1..20: mol_type = other RNA
gcgaacaagtgctacttccc

SEQ ID NO: 11984 - RNA, 20 nt, synthetic construct
  source 1..20: mol_type = other RNA
acttgttcgctggccgcccc

SEQ ID NO: 11985 - RNA, 20 nt, synthetic construct
  source 1..20: mol_type = other RNA
tgttcgctggccgcccctgg

SEQ ID NO: 11986 - RNA, 20 nt, synthetic construct
  source 1..20: mol_type = other RNA
cccctggaggctagaagctc

SEQ ID NO: 11987 - RNA, 20 nt, synthetic construct
  source 1..20: mol_type = other RNA
gagcttctagcctccagggg

SEQ ID NO: 11988 - RNA, 20 nt, synthetic construct
  source 1..20: mol_type = other RNA
ccggagcttctagcctccag

SEQ ID NO: 11989 - RNA, 20 nt, synthetic construct
  source 1..20: mol_type = other RNA
gccggagcttctagcctcca

SEQ ID NO: 11990 - RNA, 20 nt, synthetic construct
  source 1..20: mol_type = other RNA
cgccggagcttctagcctcc

SEQ ID NO: 11991 - RNA, 20 nt, synthetic construct
  source 1..20: mol_type = other RNA
agaagctccggcgccgagag

SEQ ID NO: 11992 - RNA, 20 nt, synthetic construct
  source 1..20: mol_type = other RNA
gaagctccggcgccgagagt

SEQ ID NO: 11993 - RNA, 20 nt, synthetic construct
  source 1..20: mol_type = other RNA
tccggcgccgagagtgggca

SEQ ID NO: 11994 - RNA, 20 nt, synthetic construct
  source 1..20: mol_type = other RNA
gccatgcccactctcggcgc

SEQ ID NO: 11995 - RNA, 20 nt, synthetic construct
  source 1..20: mol_type = other RNA
cgagagtgggcatggcgact

SEQ ID NO: 11996 - RNA, 20 nt, synthetic construct
  source 1..20: mol_type = other RNA
caagtcgccatgcccactct

SEQ ID NO: 11997 - RNA, 20 nt, synthetic construct
  source 1..20: mol_type = other RNA
catggcgacttggtctcagc

SEQ ID NO: 11998 - RNA, 20 nt, synthetic construct
  source 1..20: mol_type = other RNA
gacttggtctcagccggact

SEQ ID NO: 11999 - RNA, 20 nt, synthetic construct
  source 1..20: mol_type = other RNA
acttggtctcagccggactc

SEQ ID NO: 12000 - RNA, 20 nt, synthetic construct
  source 1..20: mol_type = other RNA
ctcagccggactcgggtatc

SEQ ID NO: 12001 - RNA, 20 nt, synthetic construct
  source 1..20: mol_type = other RNA
tcagccggactcgggtatcc

SEQ ID NO: 12002 - RNA, 20 nt, synthetic construct
  source 1..20: mol_type = other RNA
ccggactcgggtatccgggc

SEQ ID NO: 12003 - RNA, 20 nt, synthetic construct
  source 1..20: mol_type = other RNA
cggactcgggtatccgggca

SEQ ID NO: 12004 - RNA, 20 nt, synthetic construct
  source 1..20: mol_type = other RNA
actcgggtatccgggcaggg

SEQ ID NO: 12005 - RNA, 20 nt, synthetic construct
  source 1..20: mol_type = other RNA
cctgcccggatacccgagtc

SEQ ID NO: 12006 - RNA, 20 nt, synthetic construct
  source 1..20: mol_type = other RNA
ggcagggtgggaccagcctc

SEQ ID NO: 12007 - RNA, 20 nt, synthetic construct
  source 1..20: mol_type = other RNA
gaggctggtcccaccctgcc

SEQ ID NO: 12008 - RNA, 20 nt, synthetic construct
  source 1..20: mol_type = other RNA
gtgggaccagcctcaggcta

SEQ ID NO: 12009 - RNA, 20 nt, synthetic construct
  source 1..20: mol_type = other RNA
tgggaccagcctcaggctat

SEQ ID NO: 12010 - RNA, 20 nt, synthetic construct
  source 1..20: mol_type = other RNA
cagggcccatagcctgaggc

SEQ ID NO: 12011 - RNA, 20 nt, synthetic construct
  source 1..20: mol_type = other RNA
ggtgcagggcccatagcctg

SEQ ID NO: 12012 - RNA, 20 nt, synthetic construct
  source 1..20: mol_type = other RNA
ctgcacctacttgattttta

SEQ ID NO: 12013 - RNA, 20 nt, synthetic construct
  source 1..20: mol_type = other RNA
tgcacctacttgatttttaa

SEQ ID NO: 12014 - RNA, 20 nt, synthetic construct
  source 1..20: mol_type = other RNA
ttaaaaatcaagtaggtgca

SEQ ID NO: 12015 - RNA, 20 nt, synthetic construct
  source 1..20: mol_type = other RNA
cttaaaaatcaagtaggtgc

SEQ ID NO: 12016 - RNA, 20 nt, synthetic construct
  source 1..20: mol_type = other RNA
aagtcccttaaaaatcaagt

SEQ ID NO: 12017 - RNA, 20 nt, synthetic construct
  source 1..20: mol_type = other RNA
gatttttaagggactttgtc

SEQ ID NO: 12018 - RNA, 20 nt, synthetic construct
  source 1..20: mol_type = other RNA
tccggttcctcgaacttaat

SEQ ID NO: 12019 - RNA, 20 nt, synthetic construct
  source 1..20: mol_type = other RNA
gccaattaagttcgaggaac

SEQ ID NO: 12020 - RNA, 20 nt, synthetic construct
  source 1..20: mol_type = other RNA
cctcgaacttaattggctcc

SEQ ID NO: 12021 - RNA, 20 nt, synthetic construct
  source 1..20: mol_type = other RNA
ctcgaacttaattggctcct

SEQ ID NO: 12022 - RNA, 20 nt, synthetic construct
  source 1..20: mol_type = other RNA
gaacttaattggctcctggg

SEQ ID NO: 12023 - RNA, 20 nt, synthetic construct
  source 1..20: mol_type = other RNA
ccaggagccaattaagttcg

SEQ ID NO: 12024 - RNA, 20 nt, synthetic construct
  source 1..20: mol_type = other RNA
atttattactaaaacctccc

SEQ ID NO: 12025 - RNA, 20 nt, synthetic construct
  source 1..20: mol_type = other RNA
aaggtagaaaacacattcaa

SEQ ID NO: 12026 - RNA, 20 nt, synthetic construct
  source 1..20: mol_type = other RNA
ttttctaccttctactgtga

SEQ ID NO: 12027 - RNA, 20 nt, synthetic construct
  source 1..20: mol_type = other RNA
aggaaaaccttcacagtaga

SEQ ID NO: 12028 - RNA, 20 nt, synthetic construct
  source 1..20: mol_type = other RNA
tttcacatcatgatcagggt

SEQ ID NO: 12029 - RNA, 20 nt, synthetic construct
  source 1..20: mol_type = other RNA
tgatcatgatgtgaaaagta

SEQ ID NO: 12030 - RNA, 20 nt, synthetic construct
  source 1..20: mol_type = other RNA
tacttttcacatcatgatca

SEQ ID NO: 12031 - RNA, 20 nt, synthetic construct
  source 1..20: mol_type = other RNA
atacttttcacatcatgatc

SEQ ID NO: 12032 - RNA, 20 nt, synthetic construct
  source 1..20: mol_type = other RNA
atgggaatcacaaaagcaac

SEQ ID NO: 12033 - RNA, 20 nt, synthetic construct
  source 1..20: mol_type = other RNA
gcttttgtgattcccatttc

SEQ ID NO: 12034 - RNA, 20 nt, synthetic construct
  source 1..20: mol_type = other RNA
attcccatttcaggtttctc

SEQ ID NO: 12035 - RNA, 20 nt, synthetic construct
  source 1..20: mol_type = other RNA
tttccagagaaacctgaaat

SEQ ID NO: 12036 - RNA, 20 nt, synthetic construct
  source 1..20: mol_type = other RNA
gtttccagagaaacctgaaa

SEQ ID NO: 12037 - RNA, 20 nt, synthetic construct
  source 1..20: mol_type = other RNA
ggtttctctggaaacccccc

SEQ ID NO: 12038 - RNA, 20 nt, synthetic construct
  source 1..20: mol_type = other RNA
ggaaacccccctggtaagtg

SEQ ID NO: 12039 - RNA, 20 nt, synthetic construct
  source 1..20: mol_type = other RNA
aacccccctggtaagtgtgg

SEQ ID NO: 12040 - RNA, 20 nt, synthetic construct
  source 1..20: mol_type = other RNA
ccccctggtaagtgtggagg

SEQ ID NO: 12041 - RNA, 20 nt, synthetic construct
  source 1..20: mol_type = other RNA
cctggtaagtgtggaggagg

SEQ ID NO: 12042 - RNA, 20 nt, synthetic construct
  source 1..20: mol_type = other RNA
ctggtaagtgtggaggaggc

SEQ ID NO: 12043 - RNA, 20 nt, synthetic construct
  source 1..20: mol_type = other RNA
cctcctccacacttaccagg

SEQ ID NO: 12044 - RNA, 20 nt, synthetic construct
  source 1..20: mol_type = other RNA
gcctcctccacacttaccag

SEQ ID NO: 12045 - RNA, 20 nt, synthetic construct
  source 1..20: mol_type = other RNA
cgcctcctccacacttacca

SEQ ID NO: 12046 - RNA, 20 nt, synthetic construct
  source 1..20: mol_type = other RNA
ccgcctcctccacacttacc

SEQ ID NO: 12047 - RNA, 20 nt, synthetic construct
  source 1..20: mol_type = other RNA
acactctgacccaagacgaa

SEQ ID NO: 12048 - RNA, 20 nt, synthetic construct
  source 1..20: mol_type = other RNA
agctacaggcctttcgtctt

SEQ ID NO: 12049 - RNA, 20 nt, synthetic construct
  source 1..20: mol_type = other RNA
gagctacaggcctttcgtct

SEQ ID NO: 12050 - RNA, 20 nt, synthetic construct
  source 1..20: mol_type = other RNA
ttttctttggctggagctac

SEQ ID NO: 12051 - RNA, 20 nt, synthetic construct
  source 1..20: mol_type = other RNA
agccaaagaaaataaacctt

SEQ ID NO: 12052 - RNA, 20 nt, synthetic construct
  source 1..20: mol_type = other RNA
caaagaaaataaaccttagg

SEQ ID NO: 12053 - RNA, 20 nt, synthetic construct
  source 1..20: mol_type = other RNA
aaagaaaataaaccttagga

SEQ ID NO: 12054 - RNA, 20 nt, synthetic construct
  source 1..20: mol_type = other RNA
ctcctaaggtttattttctt

SEQ ID NO: 12055 - RNA, 20 nt, synthetic construct
  source 1..20: mol_type = other RNA
aataaaccttaggagggaga

SEQ ID NO: 12056 - RNA, 20 nt, synthetic construct
  source 1..20: mol_type = other RNA
ttttttccttctccctccta

SEQ ID NO: 12057 - RNA, 20 nt, synthetic construct
  source 1..20: mol_type = other RNA
ctgttctcaggaacagctga

SEQ ID NO: 12058 - RNA, 20 nt, synthetic construct
  source 1..20: mol_type = other RNA
ttcctgagaacagcctgcat

SEQ ID NO: 12059 - RNA, 20 nt, synthetic construct
  source 1..20: mol_type = other RNA
ttccaatgcaggctgttctc

SEQ ID NO: 12060 - RNA, 20 nt, synthetic construct
  source 1..20: mol_type = other RNA
ctgcattggaatctacagag

SEQ ID NO: 12061 - RNA, 20 nt, synthetic construct
  source 1..20: mol_type = other RNA
ctctctgtagattccaatgc

SEQ ID NO: 12062 - RNA, 20 nt, synthetic construct
  source 1..20: mol_type = other RNA
gaggacaactaatgtgagtg

SEQ ID NO: 12063 - RNA, 20 nt, synthetic construct
  source 1..20: mol_type = other RNA
agtgaggaagtgactgtatg

SEQ ID NO: 12064 - RNA, 20 nt, synthetic construct
  source 1..20: mol_type = other RNA
aagtgactgtatgtggactg

SEQ ID NO: 12065 - RNA, 20 nt, synthetic construct
  source 1..20: mol_type = other RNA
tgtggagaaagtaagtcacg

SEQ ID NO: 12066 - RNA, 20 nt, synthetic construct
  source 1..20: mol_type = other RNA
gtggagaaagtaagtcacgt

SEQ ID NO: 12067 - RNA, 20 nt, synthetic construct
  source 1..20: mol_type = other RNA
gtaagtcacgtgggcccttg

SEQ ID NO: 12068 - RNA, 20 nt, synthetic construct
  source 1..20: mol_type = other RNA
cacgtgggcccttgaggacc

SEQ ID NO: 12069 - RNA, 20 nt, synthetic construct
  source 1..20: mol_type = other RNA
gggcccttgaggacctggac

SEQ ID NO: 12070 - RNA, 20 nt, synthetic construct
  source 1..20: mol_type = other RNA
ggcccttgaggacctggact

SEQ ID NO: 12071 - RNA, 20 nt, synthetic construct
  source 1..20: mol_type = other RNA
ttgaggacctggactgggtt

SEQ ID NO: 12072 - RNA, 20 nt, synthetic construct
  source 1..20: mol_type = other RNA
aacccagtccaggtcctcaa

SEQ ID NO: 12073 - RNA, 20 nt, synthetic construct
  source 1..20: mol_type = other RNA
taacccagtccaggtcctca

SEQ ID NO: 12074 - RNA, 20 nt, synthetic construct
  source 1..20: mol_type = other RNA
aactgttcctaacccagtcc

SEQ ID NO: 12075 - RNA, 20 nt, synthetic construct
  source 1..20: mol_type = other RNA
aggaacagttgtactttcag

SEQ ID NO: 12076 - RNA, 20 nt, synthetic construct
  source 1..20: mol_type = other RNA
cagttgtactttcagaggtg

SEQ ID NO: 12077 - RNA, 20 nt, synthetic construct
  source 1..20: mol_type = other RNA
tcagaggtgaggtgtcgaga

SEQ ID NO: 12078 - RNA, 20 nt, synthetic construct
  source 1..20: mol_type = other RNA
cagaggtgaggtgtcgagaa

SEQ ID NO: 12079 - RNA, 20 nt, synthetic construct
  source 1..20: mol_type = other RNA
tcgagaagggaaagtgaatg

SEQ ID NO: 12080 - RNA, 20 nt, synthetic construct
  source 1..20: mol_type = other RNA
aagggaaagtgaatgtggtc

SEQ ID NO: 12081 - RNA, 20 nt, synthetic construct
  source 1..20: mol_type = other RNA
tgtggtctggagtgtgtcct

SEQ ID NO: 12082 - RNA, 20 nt, synthetic construct
  source 1..20: mol_type = other RNA
ctggagtgtgtccttggcct

SEQ ID NO: 12083 - RNA, 20 nt, synthetic construct
  source 1..20: mol_type = other RNA
gtccttggccttggctccac

SEQ ID NO: 12084 - RNA, 20 nt, synthetic construct
  source 1..20: mol_type = other RNA
tccttggccttggctccaca

SEQ ID NO: 12085 - RNA, 20 nt, synthetic construct
  source 1..20: mol_type = other RNA
accctgtggagccaaggcca

SEQ ID NO: 12086 - RNA, 20 nt, synthetic construct
  source 1..20: mol_type = other RNA
aagcacaccctgtggagcca

SEQ ID NO: 12087 - RNA, 20 nt, synthetic construct
  source 1..20: mol_type = other RNA
ccacagggtgtgctttcctc

SEQ ID NO: 12088 - RNA, 20 nt, synthetic construct
  source 1..20: mol_type = other RNA
cacagggtgtgctttcctct

SEQ ID NO: 12089 - RNA, 20 nt, synthetic construct
  source 1..20: mol_type = other RNA
acagggtgtgctttcctctg

SEQ ID NO: 12090 - RNA, 20 nt, synthetic construct
  source 1..20: mol_type = other RNA
ccagaggaaagcacaccctg

SEQ ID NO: 12091 - RNA, 20 nt, synthetic construct
  source 1..20: mol_type = other RNA
tgctttcctctggggccgtc

SEQ ID NO: 12092 - RNA, 20 nt, synthetic construct
  source 1..20: mol_type = other RNA
gctttcctctggggccgtca

SEQ ID NO: 12093 - RNA, 20 nt, synthetic construct
  source 1..20: mol_type = other RNA
gagctccctgacggccccag

SEQ ID NO: 12094 - RNA, 20 nt, synthetic construct
  source 1..20: mol_type = other RNA
acaagggatgagctccctga

SEQ ID NO: 12095 - RNA, 20 nt, synthetic construct
  source 1..20: mol_type = other RNA
ctcatcccttgtgttctgcc

SEQ ID NO: 12096 - RNA, 20 nt, synthetic construct
  source 1..20: mol_type = other RNA
tcatcccttgtgttctgcca

SEQ ID NO: 12097 - RNA, 20 nt, synthetic construct
  source 1..20: mol_type = other RNA
tcccttgtgttctgccaggg

SEQ ID NO: 12098 - RNA, 20 nt, synthetic construct
  source 1..20: mol_type = other RNA
cccttgtgttctgccagggt

SEQ ID NO: 12099 - RNA, 20 nt, synthetic construct
  source 1..20: mol_type = other RNA
ccttgtgttctgccagggtg

SEQ ID NO: 12100 - RNA, 20 nt, synthetic construct
  source 1..20: mol_type = other RNA
cccaccctggcagaacacaa

SEQ ID NO: 12101 - RNA, 20 nt, synthetic construct
  source 1..20: mol_type = other RNA
ccccaccctggcagaacaca

SEQ ID NO: 12102 - RNA, 20 nt, synthetic construct
  source 1..20: mol_type = other RNA
gttctgccagggtggggtac

SEQ ID NO: 12103 - RNA, 20 nt, synthetic construct
  source 1..20: mol_type = other RNA
ttctgccagggtggggtacg

SEQ ID NO: 12104 - RNA, 20 nt, synthetic construct
  source 1..20: mol_type = other RNA
tcaaaccccgtaccccaccc

SEQ ID NO: 12105 - RNA, 20 nt, synthetic construct
  source 1..20: mol_type = other RNA
gggtacggggtttgacactg

SEQ ID NO: 12106 - RNA, 20 nt, synthetic construct
  source 1..20: mol_type = other RNA
tacggggtttgacactgagg

SEQ ID NO: 12107 - RNA, 20 nt, synthetic construct
  source 1..20: mol_type = other RNA
acggggtttgacactgagga

SEQ ID NO: 12108 - RNA, 20 nt, synthetic construct
  source 1..20: mol_type = other RNA
cactgaggagggtaacctgc

SEQ ID NO: 12109 - RNA, 20 nt, synthetic construct
  source 1..20: mol_type = other RNA
gaggagggtaacctgctggc

SEQ ID NO: 12110 - RNA, 20 nt, synthetic construct
  source 1..20: mol_type = other RNA
gggtaacctgctggctggag

SEQ ID NO: 12111 - RNA, 20 nt, synthetic construct
  source 1..20: mol_type = other RNA
tggctggagcggcagagcag

SEQ ID NO: 12112 - RNA, 20 nt, synthetic construct
  source 1..20: mol_type = other RNA
agtggccttgatttgtcttt

SEQ ID NO: 12113 - RNA, 20 nt, synthetic construct
  source 1..20: mol_type = other RNA
atcttccaaaagacaaatca

SEQ ID NO: 12114 - RNA, 20 nt, synthetic construct
  source 1..20: mol_type = other RNA
accaaaaagcataaacattc

SEQ ID NO: 12115 - RNA, 20 nt, synthetic construct
  source 1..20: mol_type = other RNA
accagaatgtttatgctttt

SEQ ID NO: 12116 - RNA, 20 nt, synthetic construct
  source 1..20: mol_type = other RNA
ttcagagaaagcattgctga

SEQ ID NO: 12117 - RNA, 20 nt, synthetic construct
  source 1..20: mol_type = other RNA
ttctctgaagaaatacttaa

SEQ ID NO: 12118 - RNA, 20 nt, synthetic construct
  source 1..20: mol_type = other RNA
ctgaagaaatacttaacgga

SEQ ID NO: 12119 - RNA, 20 nt, synthetic construct
  source 1..20: mol_type = other RNA
aactcagcagaatggtgaac

SEQ ID NO: 12120 - RNA, 20 nt, synthetic construct
  source 1..20: mol_type = other RNA
accattctgctgagtttgat

SEQ ID NO: 12121 - RNA, 20 nt, synthetic construct
  source 1..20: mol_type = other RNA
ccattctgctgagtttgatt

SEQ ID NO: 12122 - RNA, 20 nt, synthetic construct
  source 1..20: mol_type = other RNA
cattctgctgagtttgattg

SEQ ID NO: 12123 - RNA, 20 nt, synthetic construct
  source 1..20: mol_type = other RNA
cccaatcaaactcagcagaa

SEQ ID NO: 12124 - RNA, 20 nt, synthetic construct
  source 1..20: mol_type = other RNA
tgctgagtttgattggggta

SEQ ID NO: 12125 - RNA, 20 nt, synthetic construct
  source 1..20: mol_type = other RNA
gctgagtttgattggggtac

SEQ ID NO: 12126 - RNA, 20 nt, synthetic construct
  source 1..20: mol_type = other RNA
gagtttgattggggtacggg

SEQ ID NO: 12127 - RNA, 20 nt, synthetic construct
  source 1..20: mol_type = other RNA
gattggggtacgggtggacg

SEQ ID NO: 12128 - RNA, 20 nt, synthetic construct
  source 1..20: mol_type = other RNA
gtgggggaagctgtgaggtc

SEQ ID NO: 12129 - RNA, 20 nt, synthetic construct
  source 1..20: mol_type = other RNA
ctcacagcttcccccactcc

SEQ ID NO: 12130 - RNA, 20 nt, synthetic construct
  source 1..20: mol_type = other RNA
ccggagtgggggaagctgtg

SEQ ID NO: 12131 - RNA, 20 nt, synthetic construct
  source 1..20: mol_type = other RNA
cccactccgggagatcatcc

SEQ ID NO: 12132 - RNA, 20 nt, synthetic construct
  source 1..20: mol_type = other RNA
ccactccgggagatcatcct

SEQ ID NO: 12133 - RNA, 20 nt, synthetic construct
  source 1..20: mol_type = other RNA
cactccgggagatcatcctg

SEQ ID NO: 12134 - RNA, 20 nt, synthetic construct
  source 1..20: mol_type = other RNA
aggatgatctcccggagtgg

SEQ ID NO: 12135 - RNA, 20 nt, synthetic construct
  source 1..20: mol_type = other RNA
caggatgatctcccggagtg

SEQ ID NO: 12136 - RNA, 20 nt, synthetic construct
  source 1..20: mol_type = other RNA
ccaggatgatctcccggagt

SEQ ID NO: 12137 - RNA, 20 nt, synthetic construct
  source 1..20: mol_type = other RNA
cccaggatgatctcccggag

SEQ ID NO: 12138 - RNA, 20 nt, synthetic construct
  source 1..20: mol_type = other RNA
tgggccccaggatgatctcc

SEQ ID NO: 12139 - RNA, 20 nt, synthetic construct
  source 1..20: mol_type = other RNA
tataggcagaactgggcccc

SEQ ID NO: 12140 - RNA, 20 nt, synthetic construct
  source 1..20: mol_type = other RNA
gtctgagtataggcagaact

SEQ ID NO: 12141 - RNA, 20 nt, synthetic construct
  source 1..20: mol_type = other RNA
ggtctgagtataggcagaac

SEQ ID NO: 12142 - RNA, 20 nt, synthetic construct
  source 1..20: mol_type = other RNA
gtggaactgggtctgagtat

SEQ ID NO: 12143 - RNA, 20 nt, synthetic construct
  source 1..20: mol_type = other RNA
agacccagttccacaacctg

SEQ ID NO: 12144 - RNA, 20 nt, synthetic construct
  source 1..20: mol_type = other RNA
attcctcaggttgtggaact

SEQ ID NO: 12145 - RNA, 20 nt, synthetic construct
  source 1..20: mol_type = other RNA
tattcctcaggttgtggaac

SEQ ID NO: 12146 - RNA, 20 nt, synthetic construct
  source 1..20: mol_type = other RNA
ccacaacctgaggaatacct

SEQ ID NO: 12147 - RNA, 20 nt, synthetic construct
  source 1..20: mol_type = other RNA
aacctgaggaataccttgga

SEQ ID NO: 12148 - RNA, 20 nt, synthetic construct
  source 1..20: mol_type = other RNA
ccaaggtattcctcaggttg

SEQ ID NO: 12149 - RNA, 20 nt, synthetic construct
  source 1..20: mol_type = other RNA
aggaataccttggatggcta

SEQ ID NO: 12150 - RNA, 20 nt, synthetic construct
  source 1..20: mol_type = other RNA
agccatccaaggtattcctc

SEQ ID NO: 12151 - RNA, 20 nt, synthetic construct
  source 1..20: mol_type = other RNA
gtggataccatagccatcca

SEQ ID NO: 12152 - RNA, 20 nt, synthetic construct
  source 1..20: mol_type = other RNA
ccaccccaagagcatagacc

SEQ ID NO: 12153 - RNA, 20 nt, synthetic construct
  source 1..20: mol_type = other RNA
ccaggtctatgctcttgggg

SEQ ID NO: 12154 - RNA, 20 nt, synthetic construct
  source 1..20: mol_type = other RNA
tgtccaggtctatgctcttg

SEQ ID NO: 12155 - RNA, 20 nt, synthetic construct
  source 1..20: mol_type = other RNA
ttgtccaggtctatgctctt

SEQ ID NO: 12156 - RNA, 20 nt, synthetic construct
  source 1..20: mol_type = other RNA
attgtccaggtctatgctct

SEQ ID NO: 12157 - RNA, 20 nt, synthetic construct
  source 1..20: mol_type = other RNA
tggacaattacttcactgcc

SEQ ID NO: 12158 - RNA, 20 nt, synthetic construct
  source 1..20: mol_type = other RNA
acaattacttcactgcccgg

SEQ ID NO: 12159 - RNA, 20 nt, synthetic construct
  source 1..20: mol_type = other RNA
tgcccggcggctcctcagtc

SEQ ID NO: 12160 - RNA, 20 nt, synthetic construct
  source 1..20: mol_type = other RNA
ggcggctcctcagtcaggtg

SEQ ID NO: 12161 - RNA, 20 nt, synthetic construct
  source 1..20: mol_type = other RNA
gcggctcctcagtcaggtga

SEQ ID NO: 12162 - RNA, 20 nt, synthetic construct
  source 1..20: mol_type = other RNA
cacctgactgaggagccgcc

SEQ ID NO: 12163 - RNA, 20 nt, synthetic construct
  source 1..20: mol_type = other RNA
tcacctgactgaggagccgc

SEQ ID NO: 12164 - RNA, 20 nt, synthetic construct
  source 1..20: mol_type = other RNA
cctcagtcaggtgagggccc

SEQ ID NO: 12165 - RNA, 20 nt, synthetic construct
  source 1..20: mol_type = other RNA
ccagggccctcacctgactg

SEQ ID NO: 12166 - RNA, 20 nt, synthetic construct
  source 1..20: mol_type = other RNA
gagggccctggacaggttcc

SEQ ID NO: 12167 - RNA, 20 nt, synthetic construct
  source 1..20: mol_type = other RNA
tggcacctggaacctgtcca

SEQ ID NO: 12168 - RNA, 20 nt, synthetic construct
  source 1..20: mol_type = other RNA
ttggcacctggaacctgtcc

SEQ ID NO: 12169 - RNA, 20 nt, synthetic construct
  source 1..20: mol_type = other RNA
gttccaggtgccaaccactg

SEQ ID NO: 12170 - RNA, 20 nt, synthetic construct
  source 1..20: mol_type = other RNA
ttacctcagtggttggcacc

SEQ ID NO: 12171 - RNA, 20 nt, synthetic construct
  source 1..20: mol_type = other RNA
caaccactgaggtaaatgcc

SEQ ID NO: 12172 - RNA, 20 nt, synthetic construct
  source 1..20: mol_type = other RNA
cactgaggtaaatgcctggc

SEQ ID NO: 12173 - RNA, 20 nt, synthetic construct
  source 1..20: mol_type = other RNA
cagccaggcatttacctcag

SEQ ID NO: 12174 - RNA, 20 nt, synthetic construct
  source 1..20: mol_type = other RNA
gctggttcaccgagacccag

SEQ ID NO: 12175 - RNA, 20 nt, synthetic construct
  source 1..20: mol_type = other RNA
ctggttcaccgagacccaga

SEQ ID NO: 12176 - RNA, 20 nt, synthetic construct
  source 1..20: mol_type = other RNA
tggttcaccgagacccagag

SEQ ID NO: 12177 - RNA, 20 nt, synthetic construct
  source 1..20: mol_type = other RNA
gacccagaggggtctgtctc

SEQ ID NO: 12178 - RNA, 20 nt, synthetic construct
  source 1..20: mol_type = other RNA
agacagacccctctgggtct

SEQ ID NO: 12179 - RNA, 20 nt, synthetic construct
  source 1..20: mol_type = other RNA
tgccagagacagacccctct

SEQ ID NO: 12180 - RNA, 20 nt, synthetic construct
  source 1..20: mol_type = other RNA
ctgccagagacagacccctc

SEQ ID NO: 12181 - RNA, 20 nt, synthetic construct
  source 1..20: mol_type = other RNA
tctggcagtcagcccaactc

SEQ ID NO: 12182 - RNA, 20 nt, synthetic construct
  source 1..20: mol_type = other RNA
tcgagggcgaggcctgagtt

SEQ ID NO: 12183 - RNA, 20 nt, synthetic construct
  source 1..20: mol_type = other RNA
ctcgagggcgaggcctgagt

SEQ ID NO: 12184 - RNA, 20 nt, synthetic construct
  source 1..20: mol_type = other RNA
ctcgccctcgagagttccag

SEQ ID NO: 12185 - RNA, 20 nt, synthetic construct
  source 1..20: mol_type = other RNA
cactggaactctcgagggcg

SEQ ID NO: 12186 - RNA, 20 nt, synthetic construct
  source 1..20: mol_type = other RNA
gaggccactggaactctcga

SEQ ID NO: 12187 - RNA, 20 nt, synthetic construct
  source 1..20: mol_type = other RNA
ggaggccactggaactctcg

SEQ ID NO: 12188 - RNA, 20 nt, synthetic construct
  source 1..20: mol_type = other RNA
agtggcctccaagatgtgac

SEQ ID NO: 12189 - RNA, 20 nt, synthetic construct
  source 1..20: mol_type = other RNA
tgtcacatcttggaggccac

SEQ ID NO: 12190 - RNA, 20 nt, synthetic construct
  source 1..20: mol_type = other RNA
ctgggcctgtcacatcttgg

SEQ ID NO: 12191 - RNA, 20 nt, synthetic construct
  source 1..20: mol_type = other RNA
gatgtgacaggcccagacaa

SEQ ID NO: 12192 - RNA, 20 nt, synthetic construct
  source 1..20: mol_type = other RNA
tgtctgggcctgtcacatct

SEQ ID NO: 12193 - RNA, 20 nt, synthetic construct
  source 1..20: mol_type = other RNA
tgtgacaggcccagacaacg

SEQ ID NO: 12194 - RNA, 20 nt, synthetic construct
  source 1..20: mol_type = other RNA
tttctcgcaccccgttgtct

SEQ ID NO: 12195 - RNA, 20 nt, synthetic construct
  source 1..20: mol_type = other RNA
ctttctcgcaccccgttgtc

SEQ ID NO: 12196 - RNA, 20 nt, synthetic construct
  source 1..20: mol_type = other RNA
cggggtgcgagaaagcgaaa

SEQ ID NO: 12197 - RNA, 20 nt, synthetic construct
  source 1..20: mol_type = other RNA
gcgagaaagcgaaacggagc

SEQ ID NO: 12198 - RNA, 20 nt, synthetic construct
  source 1..20: mol_type = other RNA
cgagaaagcgaaacggagca

SEQ ID NO: 12199 - RNA, 20 nt, synthetic construct
  source 1..20: mol_type = other RNA
agcgaaacggagcagggatt

SEQ ID NO: 12200 - RNA, 20 nt, synthetic construct
  source 1..20: mol_type = other RNA
gcagggattcggtgaagatt

SEQ ID NO: 12201 - RNA, 20 nt, synthetic construct
  source 1..20: mol_type = other RNA
gggattcggtgaagatttgg

SEQ ID NO: 12202 - RNA, 20 nt, synthetic construct
  source 1..20: mol_type = other RNA
cggtgaagatttggaggatt

SEQ ID NO: 12203 - RNA, 20 nt, synthetic construct
  source 1..20: mol_type = other RNA
ggtgaagatttggaggattt

SEQ ID NO: 12204 - RNA, 20 nt, synthetic construct
  source 1..20: mol_type = other RNA
gtgaagatttggaggatttg

SEQ ID NO: 12205 - RNA, 20 nt, synthetic construct
  source 1..20: mol_type = other RNA
tgaagatttggaggatttgg

SEQ ID NO: 12206 - RNA, 20 nt, synthetic construct
  source 1..20: mol_type = other RNA
gctgtagcccccccagtcag

SEQ ID NO: 12207 - RNA, 20 nt, synthetic construct
  source 1..20: mol_type = other RNA
taagtctccactgactgggg

SEQ ID NO: 12208 - RNA, 20 nt, synthetic construct
  source 1..20: mol_type = other RNA
ttaagtctccactgactggg

SEQ ID NO: 12209 - RNA, 20 nt, synthetic construct
  source 1..20: mol_type = other RNA
gttaagtctccactgactgg

SEQ ID NO: 12210 - RNA, 20 nt, synthetic construct
  source 1..20: mol_type = other RNA
ggttaagtctccactgactg

SEQ ID NO: 12211 - RNA, 20 nt, synthetic construct
  source 1..20: mol_type = other RNA
tggttaagtctccactgact

SEQ ID NO: 12212 - RNA, 20 nt, synthetic construct
  source 1..20: mol_type = other RNA
ttggttaagtctccactgac

SEQ ID NO: 12213 - RNA, 20 nt, synthetic construct
  source 1..20: mol_type = other RNA
gacttaaccaaagaggttag

SEQ ID NO: 12214 - RNA, 20 nt, synthetic construct
  source 1..20: mol_type = other RNA
caaagaggttagtggacctg

SEQ ID NO: 12215 - RNA, 20 nt, synthetic construct
  source 1..20: mol_type = other RNA
agaggttagtggacctgtgg

SEQ ID NO: 12216 - RNA, 20 nt, synthetic construct
  source 1..20: mol_type = other RNA
cacaggtccactaacctctt

SEQ ID NO: 12217 - RNA, 20 nt, synthetic construct
  source 1..20: mol_type = other RNA
gtggacctgtggtgggtgtg

SEQ ID NO: 12218 - RNA, 20 nt, synthetic construct
  source 1..20: mol_type = other RNA
tggacctgtggtgggtgtgt

SEQ ID NO: 12219 - RNA, 20 nt, synthetic construct
  source 1..20: mol_type = other RNA
ggacctgtggtgggtgtgtg

SEQ ID NO: 12220 - RNA, 20 nt, synthetic construct
  source 1..20: mol_type = other RNA
tgtggtgggtgtgtggggcc

SEQ ID NO: 12221 - RNA, 20 nt, synthetic construct
  source 1..20: mol_type = other RNA
gtggtgggtgtgtggggcct

SEQ ID NO: 12222 - RNA, 20 nt, synthetic construct
  source 1..20: mol_type = other RNA
tggtgggtgtgtggggcctg

SEQ ID NO: 12223 - RNA, 20 nt, synthetic construct
  source 1..20: mol_type = other RNA
aggccccacacacccaccac

SEQ ID NO: 12224 - RNA, 20 nt, synthetic construct
  source 1..20: mol_type = other RNA
ggtgtgtggggcctggggct

SEQ ID NO: 12225 - RNA, 20 nt, synthetic construct
  source 1..20: mol_type = other RNA
gtgtgtggggcctggggctt

SEQ ID NO: 12226 - RNA, 20 nt, synthetic construct
  source 1..20: mol_type = other RNA
tgtgtggggcctggggcttg

SEQ ID NO: 12227 - RNA, 20 nt, synthetic construct
  source 1..20: mol_type = other RNA
gtgtggggcctggggcttgg

SEQ ID NO: 12228 - RNA, 20 nt, synthetic construct
  source 1..20: mol_type = other RNA
tggggcctggggcttggggg

SEQ ID NO: 12229 - RNA, 20 nt, synthetic construct
  source 1..20: mol_type = other RNA
ggggcctggggcttgggggt

SEQ ID NO: 12230 - RNA, 20 nt, synthetic construct
  source 1..20: mol_type = other RNA
cctggggcttgggggtgggc

SEQ ID NO: 12231 - RNA, 20 nt, synthetic construct
  source 1..20: mol_type = other RNA
ccagcccacccccaagcccc

SEQ ID NO: 12232 - RNA, 20 nt, synthetic construct
  source 1..20: mol_type = other RNA
tgggggtgggctggtcccaa

SEQ ID NO: 12233 - RNA, 20 nt, synthetic construct
  source 1..20: mol_type = other RNA
gggctggtcccaaaggattg

SEQ ID NO: 12234 - RNA, 20 nt, synthetic construct
  source 1..20: mol_type = other RNA
tgttctgaccacaatccttt

SEQ ID NO: 12235 - RNA, 20 nt, synthetic construct
  source 1..20: mol_type = other RNA
gtgttctgaccacaatcctt

SEQ ID NO: 12236 - RNA, 20 nt, synthetic construct
  source 1..20: mol_type = other RNA
agccctgtaaagagccagac

SEQ ID NO: 12237 - RNA, 20 nt, synthetic construct
  source 1..20: mol_type = other RNA
aacctgtctggctctttaca

SEQ ID NO: 12238 - RNA, 20 nt, synthetic construct
  source 1..20: mol_type = other RNA
aaacctgtctggctctttac

SEQ ID NO: 12239 - RNA, 20 nt, synthetic construct
  source 1..20: mol_type = other RNA
agagccagacaggtttcagc

SEQ ID NO: 12240 - RNA, 20 nt, synthetic construct
  source 1..20: mol_type = other RNA
gagccagacaggtttcagca

SEQ ID NO: 12241 - RNA, 20 nt, synthetic construct
  source 1..20: mol_type = other RNA
acaggtttcagcagggcctc

SEQ ID NO: 12242 - RNA, 20 nt, synthetic construct
  source 1..20: mol_type = other RNA
aggccctgctgaaacctgtc

SEQ ID NO: 12243 - RNA, 20 nt, synthetic construct
  source 1..20: mol_type = other RNA
agctgggaggggccccaccc

SEQ ID NO: 12244 - RNA, 20 nt, synthetic construct
  source 1..20: mol_type = other RNA
gggccccacccaggactaac

SEQ ID NO: 12245 - RNA, 20 nt, synthetic construct
  source 1..20: mol_type = other RNA
ggccccacccaggactaact

SEQ ID NO: 12246 - RNA, 20 nt, synthetic construct
  source 1..20: mol_type = other RNA
gccccacccaggactaactg

SEQ ID NO: 12247 - RNA, 20 nt, synthetic construct
  source 1..20: mol_type = other RNA
accccagttagtcctgggtg

SEQ ID NO: 12248 - RNA, 20 nt, synthetic construct
  source 1..20: mol_type = other RNA
caccccagttagtcctgggt

SEQ ID NO: 12249 - RNA, 20 nt, synthetic construct
  source 1..20: mol_type = other RNA
tcaccccagttagtcctggg

SEQ ID NO: 12250 - RNA, 20 nt, synthetic construct
  source 1..20: mol_type = other RNA
ggactaactggggtgacact

SEQ ID NO: 12251 - RNA, 20 nt, synthetic construct
  source 1..20: mol_type = other RNA
gtgtcaccccagttagtcct

SEQ ID NO: 12252 - RNA, 20 nt, synthetic construct
  source 1..20: mol_type = other RNA
agtgtcaccccagttagtcc

SEQ ID NO: 12253 - RNA, 20 nt, synthetic construct
  source 1..20: mol_type = other RNA
ctaactggggtgacactagg

SEQ ID NO: 12254 - RNA, 20 nt, synthetic construct
  source 1..20: mol_type = other RNA
taactggggtgacactagga

SEQ ID NO: 12255 - RNA, 20 nt, synthetic construct
  source 1..20: mol_type = other RNA
gacactaggagggaactctg

SEQ ID NO: 12256 - RNA, 20 nt, synthetic construct
  source 1..20: mol_type = other RNA
acactaggagggaactctga

SEQ ID NO: 12257 - RNA, 20 nt, synthetic construct
  source 1..20: mol_type = other RNA
cactaggagggaactctgag

SEQ ID NO: 12258 - RNA, 20 nt, synthetic construct
  source 1..20: mol_type = other RNA
aggagggaactctgaggggc

SEQ ID NO: 12259 - RNA, 20 nt, synthetic construct
  source 1..20: mol_type = other RNA
gaactctgaggggcaggaca

SEQ ID NO: 12260 - RNA, 20 nt, synthetic construct
  source 1..20: mol_type = other RNA
tctgaggggcaggacaagga

SEQ ID NO: 12261 - RNA, 20 nt, synthetic construct
  source 1..20: mol_type = other RNA
ctgaggggcaggacaaggaa

SEQ ID NO: 12262 - RNA, 20 nt, synthetic construct
  source 1..20: mol_type = other RNA
gcaggacaaggaagggacct

SEQ ID NO: 12263 - RNA, 20 nt, synthetic construct
  source 1..20: mol_type = other RNA
caggacaaggaagggacctt

SEQ ID NO: 12264 - RNA, 20 nt, synthetic construct
  source 1..20: mol_type = other RNA
actttagctctaagatccca

SEQ ID NO: 12265 - RNA, 20 nt, synthetic construct
  source 1..20: mol_type = other RNA
agtcatgtgatctgtctttc

SEQ ID NO: 12266 - RNA, 20 nt, synthetic construct
  source 1..20: mol_type = other RNA
tagatctgattgacatcctt

SEQ ID NO: 12267 - RNA, 20 nt, synthetic construct
  source 1..20: mol_type = other RNA
gattgacatcctttggcgac

SEQ ID NO: 12268 - RNA, 20 nt, synthetic construct
  source 1..20: mol_type = other RNA
ttggcgacaggatattgatc

SEQ ID NO: 12269 - RNA, 20 nt, synthetic construct
  source 1..20: mol_type = other RNA
tggcgacaggatattgatct

SEQ ID NO: 12270 - RNA, 20 nt, synthetic construct
  source 1..20: mol_type = other RNA
gatcaatatcctgtcgccaa

SEQ ID NO: 12271 - RNA, 20 nt, synthetic construct
  source 1..20: mol_type = other RNA
gcgacaggatattgatctgg

SEQ ID NO: 12272 - RNA, 20 nt, synthetic construct
  source 1..20: mol_type = other RNA
caggatattgatctgggggc

SEQ ID NO: 12273 - RNA, 20 nt, synthetic construct
  source 1..20: mol_type = other RNA
aggatattgatctgggggct

SEQ ID NO: 12274 - RNA, 20 nt, synthetic construct
  source 1..20: mol_type = other RNA
tgatctgggggctgggcgtg

SEQ ID NO: 12275 - RNA, 20 nt, synthetic construct
  source 1..20: mol_type = other RNA
tgactatagtcaccgccaga

SEQ ID NO: 12276 - RNA, 20 nt, synthetic construct
  source 1..20: mol_type = other RNA
tagtcaccgccagaaggagc

SEQ ID NO: 12277 - RNA, 20 nt, synthetic construct
  source 1..20: mol_type = other RNA
ccgccagaaggagcaggatg

SEQ ID NO: 12278 - RNA, 20 nt, synthetic construct
  source 1..20: mol_type = other RNA
ccacatcctgctccttctgg

SEQ ID NO: 12279 - RNA, 20 nt, synthetic construct
  source 1..20: mol_type = other RNA
gaaggagcaggatgtggaga

SEQ ID NO: 12280 - RNA, 20 nt, synthetic construct
  source 1..20: mol_type = other RNA
tctccacatcctgctccttc

SEQ ID NO: 12281 - RNA, 20 nt, synthetic construct
  source 1..20: mol_type = other RNA
gtggagaaggagctgcgaga

SEQ ID NO: 12282 - RNA, 20 nt, synthetic construct
  source 1..20: mol_type = other RNA
gagaaggagctgcgagatgg

SEQ ID NO: 12283 - RNA, 20 nt, synthetic construct
  source 1..20: mol_type = other RNA
gctgcgagatggaggcgagc

SEQ ID NO: 12284 - RNA, 20 nt, synthetic construct
  source 1..20: mol_type = other RNA
atggaggcgagcaggacacc

SEQ ID NO: 12285 - RNA, 20 nt, synthetic construct
  source 1..20: mol_type = other RNA
tggaggcgagcaggacacct

SEQ ID NO: 12286 - RNA, 20 nt, synthetic construct
  source 1..20: mol_type = other RNA
ggcgagcaggacacctgggc

SEQ ID NO: 12287 - RNA, 20 nt, synthetic construct
  source 1..20: mol_type = other RNA
gcaggacacctgggcaggcg

SEQ ID NO: 12288 - RNA, 20 nt, synthetic construct
  source 1..20: mol_type = other RNA
caggacacctgggcaggcga

SEQ ID NO: 12289 - RNA, 20 nt, synthetic construct
  source 1..20: mol_type = other RNA
cacctgggcaggcgagggcg

SEQ ID NO: 12290 - RNA, 20 nt, synthetic construct
  source 1..20: mol_type = other RNA
ttccgcgccctcgcctgccc

SEQ ID NO: 12291 - RNA, 20 nt, synthetic construct
  source 1..20: mol_type = other RNA
aggcgagggcgcggaagctc

SEQ ID NO: 12292 - RNA, 20 nt, synthetic construct
  source 1..20: mol_type = other RNA
agggcgcggaagctctggca

SEQ ID NO: 12293 - RNA, 20 nt, synthetic construct
  source 1..20: mol_type = other RNA
tctggcacggaacctgctag

SEQ ID NO: 12294 - RNA, 20 nt, synthetic construct
  source 1..20: mol_type = other RNA
gcacggaacctgctagtgga

SEQ ID NO: 12295 - RNA, 20 nt, synthetic construct
  source 1..20: mol_type = other RNA
ctgctagtggatggagagac

SEQ ID NO: 12296 - RNA, 20 nt, synthetic construct
  source 1..20: mol_type = other RNA
tgctagtggatggagagact

SEQ ID NO: 12297 - RNA, 20 nt, synthetic construct
  source 1..20: mol_type = other RNA
gctagtggatggagagactg

SEQ ID NO: 12298 - RNA, 20 nt, synthetic construct
  source 1..20: mol_type = other RNA
cagtctctccatccactagc

SEQ ID NO: 12299 - RNA, 20 nt, synthetic construct
  source 1..20: mol_type = other RNA
tggggagagcttccctgcac

SEQ ID NO: 12300 - RNA, 20 nt, synthetic construct
  source 1..20: mol_type = other RNA
ggggcgatggtacctgtgca

SEQ ID NO: 12301 - RNA, 20 nt, synthetic construct
  source 1..20: mol_type = other RNA
aggggcgatggtacctgtgc

SEQ ID NO: 12302 - RNA, 20 nt, synthetic construct
  source 1..20: mol_type = other RNA
gtaccatcgcccctgctcac

SEQ ID NO: 12303 - RNA, 20 nt, synthetic construct
  source 1..20: mol_type = other RNA
taccatcgcccctgctcact

SEQ ID NO: 12304 - RNA, 20 nt, synthetic construct
  source 1..20: mol_type = other RNA
agcccagtgagcaggggcga

SEQ ID NO: 12305 - RNA, 20 nt, synthetic construct
  source 1..20: mol_type = other RNA
gaagagagcccagtgagcag

SEQ ID NO: 12306 - RNA, 20 nt, synthetic construct
  source 1..20: mol_type = other RNA
agaagagagcccagtgagca

SEQ ID NO: 12307 - RNA, 20 nt, synthetic construct
  source 1..20: mol_type = other RNA
aagaagagagcccagtgagc

SEQ ID NO: 12308 - RNA, 20 nt, synthetic construct
  source 1..20: mol_type = other RNA
ctactaccctgacacaaacc

SEQ ID NO: 12309 - RNA, 20 nt, synthetic construct
  source 1..20: mol_type = other RNA
tggtttgtgtcagggtagta

SEQ ID NO: 12310 - RNA, 20 nt, synthetic construct
  source 1..20: mol_type = other RNA
ctggtttgtgtcagggtagt

SEQ ID NO: 12311 - RNA, 20 nt, synthetic construct
  source 1..20: mol_type = other RNA
ctccagcctggtttgtgtca

SEQ ID NO: 12312 - RNA, 20 nt, synthetic construct
  source 1..20: mol_type = other RNA
actccagcctggtttgtgtc

SEQ ID NO: 12313 - RNA, 20 nt, synthetic construct
  source 1..20: mol_type = other RNA
tttctggaagaactccagcc

SEQ ID NO: 12314 - RNA, 20 nt, synthetic construct
  source 1..20: mol_type = other RNA
aaacttcctttagagaagac

SEQ ID NO: 12315 - RNA, 20 nt, synthetic construct
  source 1..20: mol_type = other RNA
tcttctctaaaggaagtttc

SEQ ID NO: 12316 - RNA, 20 nt, synthetic construct
  source 1..20: mol_type = other RNA
cttcctttagagaagacagg

SEQ ID NO: 12317 - RNA, 20 nt, synthetic construct
  source 1..20: mol_type = other RNA
tagagaagacaggtggtgtg

SEQ ID NO: 12318 - RNA, 20 nt, synthetic construct
  source 1..20: mol_type = other RNA
acaccacctgtcttctctaa

SEQ ID NO: 12319 - RNA, 20 nt, synthetic construct
  source 1..20: mol_type = other RNA
gagaagacaggtggtgtgtg

SEQ ID NO: 12320 - RNA, 20 nt, synthetic construct
  source 1..20: mol_type = other RNA
aagacaggtggtgtgtgggg

SEQ ID NO: 12321 - RNA, 20 nt, synthetic construct
  source 1..20: mol_type = other RNA
gccagccattagcctgggaa

SEQ ID NO: 12322 - RNA, 20 nt, synthetic construct
  source 1..20: mol_type = other RNA
ccagccattagcctgggaat

SEQ ID NO: 12323 - RNA, 20 nt, synthetic construct
  source 1..20: mol_type = other RNA
gccattagcctgggaatggg

SEQ ID NO: 12324 - RNA, 20 nt, synthetic construct
  source 1..20: mol_type = other RNA
ccattagcctgggaatggga

SEQ ID NO: 12325 - RNA, 20 nt, synthetic construct
  source 1..20: mol_type = other RNA
cccattcccaggctaatggc

SEQ ID NO: 12326 - RNA, 20 nt, synthetic construct
  source 1..20: mol_type = other RNA
ccctcccattcccaggctaa

SEQ ID NO: 12327 - RNA, 20 nt, synthetic construct
  source 1..20: mol_type = other RNA
gggaatgggagggagactgc

SEQ ID NO: 12328 - RNA, 20 nt, synthetic construct
  source 1..20: mol_type = other RNA
ggaatgggagggagactgca

SEQ ID NO: 12329 - RNA, 20 nt, synthetic construct
  source 1..20: mol_type = other RNA
gcagtctccctcccattccc

SEQ ID NO: 12330 - RNA, 20 nt, synthetic construct
  source 1..20: mol_type = other RNA
ctgcagggcttcagccattc

SEQ ID NO: 12331 - RNA, 20 nt, synthetic construct
  source 1..20: mol_type = other RNA
tgcagggcttcagccattct

SEQ ID NO: 12332 - RNA, 20 nt, synthetic construct
  source 1..20: mol_type = other RNA
ctgaagcttctttcccagaa

SEQ ID NO: 12333 - RNA, 20 nt, synthetic construct
  source 1..20: mol_type = other RNA
gggaaagaagcttcagcccc

SEQ ID NO: 12334 - RNA, 20 nt, synthetic construct
  source 1..20: mol_type = other RNA
gcttcagccccaggcagcca

SEQ ID NO: 12335 - RNA, 20 nt, synthetic construct
  source 1..20: mol_type = other RNA
gccccaggcagccaaggccc

SEQ ID NO: 12336 - RNA, 20 nt, synthetic construct
  source 1..20: mol_type = other RNA
acctgggccttggctgcctg

SEQ ID NO: 12337 - RNA, 20 nt, synthetic construct
  source 1..20: mol_type = other RNA
gacctgggccttggctgcct

SEQ ID NO: 12338 - RNA, 20 nt, synthetic construct
  source 1..20: mol_type = other RNA
tgacctgggccttggctgcc

SEQ ID NO: 12339 - RNA, 20 nt, synthetic construct
  source 1..20: mol_type = other RNA
agtctgattgacctgggcct

SEQ ID NO: 12340 - RNA, 20 nt, synthetic construct
  source 1..20: mol_type = other RNA
actgtaagtctgattgacct

SEQ ID NO: 12341 - RNA, 20 nt, synthetic construct
  source 1..20: mol_type = other RNA
aactgtaagtctgattgacc

SEQ ID NO: 12342 - RNA, 20 nt, synthetic construct
  source 1..20: mol_type = other RNA
cttacagttcctgttgccac

SEQ ID NO: 12343 - RNA, 20 nt, synthetic construct
  source 1..20: mol_type = other RNA
ctgttgccacaggtgcctag

SEQ ID NO: 12344 - RNA, 20 nt, synthetic construct
  source 1..20: mol_type = other RNA
tgttgccacaggtgcctagt

SEQ ID NO: 12345 - RNA, 20 nt, synthetic construct
  source 1..20: mol_type = other RNA
gttgccacaggtgcctagtg

SEQ ID NO: 12346 - RNA, 20 nt, synthetic construct
  source 1..20: mol_type = other RNA
cactaggcacctgtggcaac

SEQ ID NO: 12347 - RNA, 20 nt, synthetic construct
  source 1..20: mol_type = other RNA
gccacaggtgcctagtgggg

SEQ ID NO: 12348 - RNA, 20 nt, synthetic construct
  source 1..20: mol_type = other RNA
tcctccccactaggcacctg

SEQ ID NO: 12349 - RNA, 20 nt, synthetic construct
  source 1..20: mol_type = other RNA
gcctagtggggaggaccaga

SEQ ID NO: 12350 - RNA, 20 nt, synthetic construct
  source 1..20: mol_type = other RNA
gccgtctggtcctccccact

SEQ ID NO: 12351 - RNA, 20 nt, synthetic construct
  source 1..20: mol_type = other RNA
ggaccagacggccctgtccc

SEQ ID NO: 12352 - RNA, 20 nt, synthetic construct
  source 1..20: mol_type = other RNA
cttccagggacagggccgtc

SEQ ID NO: 12353 - RNA, 20 nt, synthetic construct
  source 1..20: mol_type = other RNA
tgtccctggaagagtgcctt

SEQ ID NO: 12354 - RNA, 20 nt, synthetic construct
  source 1..20: mol_type = other RNA
aaggcactcttccagggaca

SEQ ID NO: 12355 - RNA, 20 nt, synthetic construct
  source 1..20: mol_type = other RNA
taaggcactcttccagggac

SEQ ID NO: 12356 - RNA, 20 nt, synthetic construct
  source 1..20: mol_type = other RNA
ggaagagtgccttaggctgc

SEQ ID NO: 12357 - RNA, 20 nt, synthetic construct
  source 1..20: mol_type = other RNA
cagcctaaggcactcttcca

SEQ ID NO: 12358 - RNA, 20 nt, synthetic construct
  source 1..20: mol_type = other RNA
gcagcctaaggcactcttcc

SEQ ID NO: 12359 - RNA, 20 nt, synthetic construct
  source 1..20: mol_type = other RNA
aggtggcttccagcagccta

SEQ ID NO: 12360 - RNA, 20 nt, synthetic construct
  source 1..20: mol_type = other RNA
ctggaagccacctgcccctt

SEQ ID NO: 12361 - RNA, 20 nt, synthetic construct
  source 1..20: mol_type = other RNA
tggaagccacctgccccttt

SEQ ID NO: 12362 - RNA, 20 nt, synthetic construct
  source 1..20: mol_type = other RNA
ggaagccacctgcccctttg

SEQ ID NO: 12363 - RNA, 20 nt, synthetic construct
  source 1..20: mol_type = other RNA
attctccccaaaggggcagg

SEQ ID NO: 12364 - RNA, 20 nt, synthetic construct
  source 1..20: mol_type = other RNA
cccctttggggagaatgctg

SEQ ID NO: 12365 - RNA, 20 nt, synthetic construct
  source 1..20: mol_type = other RNA
agcattctccccaaaggggc

SEQ ID NO: 12366 - RNA, 20 nt, synthetic construct
  source 1..20: mol_type = other RNA
cctcagcattctccccaaag

SEQ ID NO: 12367 - RNA, 20 nt, synthetic construct
  source 1..20: mol_type = other RNA
acctcagcattctccccaaa

SEQ ID NO: 12368 - RNA, 20 nt, synthetic construct
  source 1..20: mol_type = other RNA
cacctcagcattctccccaa

SEQ ID NO: 12369 - RNA, 20 nt, synthetic construct
  source 1..20: mol_type = other RNA
gggagaatgctgaggtgagc

SEQ ID NO: 12370 - RNA, 20 nt, synthetic construct
  source 1..20: mol_type = other RNA
tgagagtccaccaagtgagc

SEQ ID NO: 12371 - RNA, 20 nt, synthetic construct
  source 1..20: mol_type = other RNA
ctcacttggtggactctcac

SEQ ID NO: 12372 - RNA, 20 nt, synthetic construct
  source 1..20: mol_type = other RNA
aggctgccctgctcacttgg

SEQ ID NO: 12373 - RNA, 20 nt, synthetic construct
  source 1..20: mol_type = other RNA
tacaggctgccctgctcact

SEQ ID NO: 12374 - RNA, 20 nt, synthetic construct
  source 1..20: mol_type = other RNA
gtacctggtgtgtccctcca

SEQ ID NO: 12375 - RNA, 20 nt, synthetic construct
  source 1..20: mol_type = other RNA
tggagggacacaccaggtac

SEQ ID NO: 12376 - RNA, 20 nt, synthetic construct
  source 1..20: mol_type = other RNA
ggtgtgtccctccatggctg

SEQ ID NO: 12377 - RNA, 20 nt, synthetic construct
  source 1..20: mol_type = other RNA
gtgtgtccctccatggctga

SEQ ID NO: 12378 - RNA, 20 nt, synthetic construct
  source 1..20: mol_type = other RNA
cagccatggagggacacacc

SEQ ID NO: 12379 - RNA, 20 nt, synthetic construct
  source 1..20: mol_type = other RNA
gctggcccctcagccatgga

SEQ ID NO: 12380 - RNA, 20 nt, synthetic construct
  source 1..20: mol_type = other RNA
atggctgaggggccagctgt

SEQ ID NO: 12381 - RNA, 20 nt, synthetic construct
  source 1..20: mol_type = other RNA
aacagctggcccctcagcca

SEQ ID NO: 12382 - RNA, 20 nt, synthetic construct
  source 1..20: mol_type = other RNA
gaggggccagctgttggttc

SEQ ID NO: 12383 - RNA, 20 nt, synthetic construct
  source 1..20: mol_type = other RNA
tgttggttctggccttattc

SEQ ID NO: 12384 - RNA, 20 nt, synthetic construct
  source 1..20: mol_type = other RNA
tctggccttattctggctgc

SEQ ID NO: 12385 - RNA, 20 nt, synthetic construct
  source 1..20: mol_type = other RNA
ctggccttattctggctgct

SEQ ID NO: 12386 - RNA, 20 nt, synthetic construct
  source 1..20: mol_type = other RNA
tggccttattctggctgctg

SEQ ID NO: 12387 - RNA, 20 nt, synthetic construct
  source 1..20: mol_type = other RNA
ggccttattctggctgctgg

SEQ ID NO: 12388 - RNA, 20 nt, synthetic construct
  source 1..20: mol_type = other RNA
tacccccagcagccagaata

SEQ ID NO: 12389 - RNA, 20 nt, synthetic construct
  source 1..20: mol_type = other RNA
gctgctgggggtaaatgcag

SEQ ID NO: 12390 - RNA, 20 nt, synthetic construct
  source 1..20: mol_type = other RNA
ctgggggtaaatgcagagga

SEQ ID NO: 12391 - RNA, 20 nt, synthetic construct
  source 1..20: mol_type = other RNA
gaggaaggaagaacagaaac

SEQ ID NO: 12392 - RNA, 20 nt, synthetic construct
  source 1..20: mol_type = other RNA
ggaagaacagaaacaggtcc

SEQ ID NO: 12393 - RNA, 20 nt, synthetic construct
  source 1..20: mol_type = other RNA
agaacagaaacaggtccagg

SEQ ID NO: 12394 - RNA, 20 nt, synthetic construct
  source 1..20: mol_type = other RNA
caggtccaggtggtaatctc

SEQ ID NO: 12395 - RNA, 20 nt, synthetic construct
  source 1..20: mol_type = other RNA
aggtccaggtggtaatctct

SEQ ID NO: 12396 - RNA, 20 nt, synthetic construct
  source 1..20: mol_type = other RNA
tccaggtggtaatctctggg

SEQ ID NO: 12397 - RNA, 20 nt, synthetic construct
  source 1..20: mol_type = other RNA
tcctcccagagattaccacc

SEQ ID NO: 12398 - RNA, 20 nt, synthetic construct
  source 1..20: mol_type = other RNA
atctctgggaggaaagcaca

SEQ ID NO: 12399 - RNA, 20 nt, synthetic construct
  source 1..20: mol_type = other RNA
agaggctttaacaaggggga

SEQ ID NO: 12400 - RNA, 20 nt, synthetic construct
  source 1..20: mol_type = other RNA
acacagaggctttaacaagg

SEQ ID NO: 12401 - RNA, 20 nt, synthetic construct
  source 1..20: mol_type = other RNA
aacacagaggctttaacaag

SEQ ID NO: 12402 - RNA, 20 nt, synthetic construct
  source 1..20: mol_type = other RNA
aaacacagaggctttaacaa

SEQ ID NO: 12403 - RNA, 20 nt, synthetic construct
  source 1..20: mol_type = other RNA
aaaacacagaggctttaaca

SEQ ID NO: 12404 - RNA, 20 nt, synthetic construct
  source 1..20: mol_type = other RNA
gaaactagggcaaaacacag

SEQ ID NO: 12405 - RNA, 20 nt, synthetic construct
  source 1..20: mol_type = other RNA
gaaatgtctgctggaaacta

SEQ ID NO: 12406 - RNA, 20 nt, synthetic construct
  source 1..20: mol_type = other RNA
ggaaatgtctgctggaaact

SEQ ID NO: 12407 - RNA, 20 nt, synthetic construct
  source 1..20: mol_type = other RNA
gttatgctggaaatgtctgc

SEQ ID NO: 12408 - RNA, 20 nt, synthetic construct
  source 1..20: mol_type = other RNA
aggcactgcttctgttatgc

SEQ ID NO: 12409 - RNA, 20 nt, synthetic construct
  source 1..20: mol_type = other RNA
gcagggggctcactctcact

SEQ ID NO: 12410 - RNA, 20 nt, synthetic construct
  source 1..20: mol_type = other RNA
aggttgttttgaagagcagg

SEQ ID NO: 12411 - RNA, 20 nt, synthetic construct
  source 1..20: mol_type = other RNA
gaggttgttttgaagagcag

SEQ ID NO: 12412 - RNA, 20 nt, synthetic construct
  source 1..20: mol_type = other RNA
agaggttgttttgaagagca

SEQ ID NO: 12413 - RNA, 20 nt, synthetic construct
  source 1..20: mol_type = other RNA
aagaggttgttttgaagagc

SEQ ID NO: 12414 - RNA, 20 nt, synthetic construct
  source 1..20: mol_type = other RNA
ctcttgtctcctcttctgac

SEQ ID NO: 12415 - RNA, 20 nt, synthetic construct
  source 1..20: mol_type = other RNA
tcttgtctcctcttctgacc

SEQ ID NO: 12416 - RNA, 20 nt, synthetic construct
  source 1..20: mol_type = other RNA
cggtcagaagaggagacaag

SEQ ID NO: 12417 - RNA, 20 nt, synthetic construct
  source 1..20: mol_type = other RNA
gactctgtcccggtcagaag

SEQ ID NO: 12418 - RNA, 20 nt, synthetic construct
  source 1..20: mol_type = other RNA
gacagagtcaccatttgatt

SEQ ID NO: 12419 - RNA, 20 nt, synthetic construct
  source 1..20: mol_type = other RNA
atcaaatggtgactctgtcc

SEQ ID NO: 12420 - RNA, 20 nt, synthetic construct
  source 1..20: mol_type = other RNA
catttgatttggaacagcag

SEQ ID NO: 12421 - RNA, 20 nt, synthetic construct
  source 1..20: mol_type = other RNA
cactgctgttccaaatcaaa

SEQ ID NO: 12422 - RNA, 20 nt, synthetic construct
  source 1..20: mol_type = other RNA
gcaagatctcatgtccatca

SEQ ID NO: 12423 - RNA, 20 nt, synthetic construct
  source 1..20: mol_type = other RNA
catgtccatcatggaaatgc

SEQ ID NO: 12424 - RNA, 20 nt, synthetic construct
  source 1..20: mol_type = other RNA
tccatcatggaaatgcaggt

SEQ ID NO: 12425 - RNA, 20 nt, synthetic construct
  source 1..20: mol_type = other RNA
tcctacctgcatttccatga

SEQ ID NO: 12426 - RNA, 20 nt, synthetic construct
  source 1..20: mol_type = other RNA
ggaaatgcaggtaggattgt

SEQ ID NO: 12427 - RNA, 20 nt, synthetic construct
  source 1..20: mol_type = other RNA
gcaggtaggattgtcggaac

SEQ ID NO: 12428 - RNA, 20 nt, synthetic construct
  source 1..20: mol_type = other RNA
caggtaggattgtcggaacc

SEQ ID NO: 12429 - RNA, 20 nt, synthetic construct
  source 1..20: mol_type = other RNA
ggaaccgggcacaaacctat

SEQ ID NO: 12430 - RNA, 20 nt, synthetic construct
  source 1..20: mol_type = other RNA
aaatccaataggtttgtgcc

SEQ ID NO: 12431 - RNA, 20 nt, synthetic construct
  source 1..20: mol_type = other RNA
caatctgtgcaaaatccaat

SEQ ID NO: 12432 - RNA, 20 nt, synthetic construct
  source 1..20: mol_type = other RNA
cagttgcttttccatctcca

SEQ ID NO: 12433 - RNA, 20 nt, synthetic construct
  source 1..20: mol_type = other RNA
acactttctctccttggaga

SEQ ID NO: 12434 - RNA, 20 nt, synthetic construct
  source 1..20: mol_type = other RNA
agtattacactttctctcct

SEQ ID NO: 12435 - RNA, 20 nt, synthetic construct
  source 1..20: mol_type = other RNA
ttccctgaatcatagagaag

SEQ ID NO: 12436 - RNA, 20 nt, synthetic construct
  source 1..20: mol_type = other RNA
tccctgaatcatagagaagt

SEQ ID NO: 12437 - RNA, 20 nt, synthetic construct
  source 1..20: mol_type = other RNA
ccctgaatcatagagaagtg

SEQ ID NO: 12438 - RNA, 20 nt, synthetic construct
  source 1..20: mol_type = other RNA
gcacagctgcatgggtgtaa

SEQ ID NO: 12439 - RNA, 20 nt, synthetic construct
  source 1..20: mol_type = other RNA
ccatgcagctgtgcctctgt

SEQ ID NO: 12440 - RNA, 20 nt, synthetic construct
  source 1..20: mol_type = other RNA
catgcagctgtgcctctgtt

SEQ ID NO: 12441 - RNA, 20 nt, synthetic construct
  source 1..20: mol_type = other RNA
caacagaggcacagctgcat

SEQ ID NO: 12442 - RNA, 20 nt, synthetic construct
  source 1..20: mol_type = other RNA
ccaacagaggcacagctgca

SEQ ID NO: 12443 - RNA, 20 nt, synthetic construct
  source 1..20: mol_type = other RNA
acactgcaggcacccaacag

SEQ ID NO: 12444 - RNA, 20 nt, synthetic construct
  source 1..20: mol_type = other RNA
gcctgcagtgtgtgagcccc

SEQ ID NO: 12445 - RNA, 20 nt, synthetic construct
  source 1..20: mol_type = other RNA
cctgcagtgtgtgagcccca

SEQ ID NO: 12446 - RNA, 20 nt, synthetic construct
  source 1..20: mol_type = other RNA
ctgcagtgtgtgagccccag

SEQ ID NO: 12447 - RNA, 20 nt, synthetic construct
  source 1..20: mol_type = other RNA
cagtgtgtgagccccagggg

SEQ ID NO: 12448 - RNA, 20 nt, synthetic construct
  source 1..20: mol_type = other RNA
ccctggggctcacacactgc

SEQ ID NO: 12449 - RNA, 20 nt, synthetic construct
  source 1..20: mol_type = other RNA
ggaactgactccctcccctg

SEQ ID NO: 12450 - RNA, 20 nt, synthetic construct
  source 1..20: mol_type = other RNA
aggaactgactccctcccct

SEQ ID NO: 12451 - RNA, 20 nt, synthetic construct
  source 1..20: mol_type = other RNA
taggaactgactccctcccc

SEQ ID NO: 12452 - RNA, 20 nt, synthetic construct
  source 1..20: mol_type = other RNA
agtcagttcctagtgaacag

SEQ ID NO: 12453 - RNA, 20 nt, synthetic construct
  source 1..20: mol_type = other RNA
gaagagcaccactgttcact

SEQ ID NO: 12454 - RNA, 20 nt, synthetic construct
  source 1..20: mol_type = other RNA
tggtgctcttctcccctccc

SEQ ID NO: 12455 - RNA, 20 nt, synthetic construct
  source 1..20: mol_type = other RNA
tcttctcccctcccaggcca

SEQ ID NO: 12456 - RNA, 20 nt, synthetic construct
  source 1..20: mol_type = other RNA
tcacttccatggcctgggag

SEQ ID NO: 12457 - RNA, 20 nt, synthetic construct
  source 1..20: mol_type = other RNA
ttcacttccatggcctggga

SEQ ID NO: 12458 - RNA, 20 nt, synthetic construct
  source 1..20: mol_type = other RNA
gttcacttccatggcctggg

SEQ ID NO: 12459 - RNA, 20 nt, synthetic construct
  source 1..20: mol_type = other RNA
tgtgttcacttccatggcct

SEQ ID NO: 12460 - RNA, 20 nt, synthetic construct
  source 1..20: mol_type = other RNA
atgtgttcacttccatggcc

SEQ ID NO: 12461 - RNA, 20 nt, synthetic construct
  source 1..20: mol_type = other RNA
tgctgatgtgttcacttcca

SEQ ID NO: 12462 - RNA, 20 nt, synthetic construct
  source 1..20: mol_type = other RNA
atcctgtacagtgcccctcc

SEQ ID NO: 12463 - RNA, 20 nt, synthetic construct
  source 1..20: mol_type = other RNA
ctccaggaggggcactgtac

SEQ ID NO: 12464 - RNA, 20 nt, synthetic construct
  source 1..20: mol_type = other RNA
gctcagtgggtctccaggag

SEQ ID NO: 12465 - RNA, 20 nt, synthetic construct
  source 1..20: mol_type = other RNA
tgctcagtgggtctccagga

SEQ ID NO: 12466 - RNA, 20 nt, synthetic construct
  source 1..20: mol_type = other RNA
gtgctcagtgggtctccagg

SEQ ID NO: 12467 - RNA, 20 nt, synthetic construct
  source 1..20: mol_type = other RNA
ttggtgctcagtgggtctcc

SEQ ID NO: 12468 - RNA, 20 nt, synthetic construct
  source 1..20: mol_type = other RNA
ggctgtagttggtgctcagt

SEQ ID NO: 12469 - RNA, 20 nt, synthetic construct
  source 1..20: mol_type = other RNA
aggctgtagttggtgctcag

SEQ ID NO: 12470 - RNA, 20 nt, synthetic construct
  source 1..20: mol_type = other RNA
gttgggggcaaggctgtagt

SEQ ID NO: 12471 - RNA, 20 nt, synthetic construct
  source 1..20: mol_type = other RNA
tgatgggagtgttgggggca

SEQ ID NO: 12472 - RNA, 20 nt, synthetic construct
  source 1..20: mol_type = other RNA
ctgattgatgggagtgttgg

SEQ ID NO: 12473 - RNA, 20 nt, synthetic construct
  source 1..20: mol_type = other RNA
tctgattgatgggagtgttg

SEQ ID NO: 12474 - RNA, 20 nt, synthetic construct
  source 1..20: mol_type = other RNA
ttctgattgatgggagtgtt

SEQ ID NO: 12475 - RNA, 20 nt, synthetic construct
  source 1..20: mol_type = other RNA
attctgattgatgggagtgt

SEQ ID NO: 12476 - RNA, 20 nt, synthetic construct
  source 1..20: mol_type = other RNA
aggctgacattctgattgat

SEQ ID NO: 12477 - RNA, 20 nt, synthetic construct
  source 1..20: mol_type = other RNA
caggctgacattctgattga

SEQ ID NO: 12478 - RNA, 20 nt, synthetic construct
  source 1..20: mol_type = other RNA
tcagaatgtcagcctgcatc

SEQ ID NO: 12479 - RNA, 20 nt, synthetic construct
  source 1..20: mol_type = other RNA
cagcctgcatcaggcgtccc

SEQ ID NO: 12480 - RNA, 20 nt, synthetic construct
  source 1..20: mol_type = other RNA
agcctgcatcaggcgtccct

SEQ ID NO: 12481 - RNA, 20 nt, synthetic construct
  source 1..20: mol_type = other RNA
gcctgcatcaggcgtccctg

SEQ ID NO: 12482 - RNA, 20 nt, synthetic construct
  source 1..20: mol_type = other RNA
cctgcatcaggcgtccctgg

SEQ ID NO: 12483 - RNA, 20 nt, synthetic construct
  source 1..20: mol_type = other RNA
ctgcatcaggcgtccctggg

SEQ ID NO: 12484 - RNA, 20 nt, synthetic construct
  source 1..20: mol_type = other RNA
cccccagggacgcctgatgc

SEQ ID NO: 12485 - RNA, 20 nt, synthetic construct
  source 1..20: mol_type = other RNA
gtccctggggggctgcagcc

SEQ ID NO: 12486 - RNA, 20 nt, synthetic construct
  source 1..20: mol_type = other RNA
gtcctggctgcagcccccca

SEQ ID NO: 12487 - RNA, 20 nt, synthetic construct
  source 1..20: mol_type = other RNA
agtcctggctgcagcccccc

SEQ ID NO: 12488 - RNA, 20 nt, synthetic construct
  source 1..20: mol_type = other RNA
ggctgaagagtaagaagtcc

SEQ ID NO: 12489 - RNA, 20 nt, synthetic construct
  source 1..20: mol_type = other RNA
cttcttactcttcagccccg

SEQ ID NO: 12490 - RNA, 20 nt, synthetic construct
  source 1..20: mol_type = other RNA
cttactcttcagccccgagg

SEQ ID NO: 12491 - RNA, 20 nt, synthetic construct
  source 1..20: mol_type = other RNA
cgaggtggaaagcctgcctg

SEQ ID NO: 12492 - RNA, 20 nt, synthetic construct
  source 1..20: mol_type = other RNA
caggcaggctttccacctcg

SEQ ID NO: 12493 - RNA, 20 nt, synthetic construct
  source 1..20: mol_type = other RNA
acaggcaggctttccacctc

SEQ ID NO: 12494 - RNA, 20 nt, synthetic construct
  source 1..20: mol_type = other RNA
cacaggcaggctttccacct

SEQ ID NO: 12495 - RNA, 20 nt, synthetic construct
  source 1..20: mol_type = other RNA
tggagctactggccacaggc

SEQ ID NO: 12496 - RNA, 20 nt, synthetic construct
  source 1..20: mol_type = other RNA
agcgtggagctactggccac

SEQ ID NO: 12497 - RNA, 20 nt, synthetic construct
  source 1..20: mol_type = other RNA
tagctccacgctgctcccgt

SEQ ID NO: 12498 - RNA, 20 nt, synthetic construct
  source 1..20: mol_type = other RNA
cgggagcagcgtggagctac

SEQ ID NO: 12499 - RNA, 20 nt, synthetic construct
  source 1..20: mol_type = other RNA
gggggccaacgggagcagcg

SEQ ID NO: 12500 - RNA, 20 nt, synthetic construct
  source 1..20: mol_type = other RNA
tagaattgctgggggccaac

SEQ ID NO: 12501 - RNA, 20 nt, synthetic construct
  source 1..20: mol_type = other RNA
gtagaattgctgggggccaa

SEQ ID NO: 12502 - RNA, 20 nt, synthetic construct
  source 1..20: mol_type = other RNA
gaggctggtagaattgctgg

SEQ ID NO: 12503 - RNA, 20 nt, synthetic construct
  source 1..20: mol_type = other RNA
tgaggctggtagaattgctg

SEQ ID NO: 12504 - RNA, 20 nt, synthetic construct
  source 1..20: mol_type = other RNA
ttgaggctggtagaattgct

SEQ ID NO: 12505 - RNA, 20 nt, synthetic construct
  source 1..20: mol_type = other RNA
gttgaggctggtagaattgc

SEQ ID NO: 12506 - RNA, 20 nt, synthetic construct
  source 1..20: mol_type = other RNA
accagcctcaactccacctt

SEQ ID NO: 12507 - RNA, 20 nt, synthetic construct
  source 1..20: mol_type = other RNA
gccgaaggtggagttgaggc

SEQ ID NO: 12508 - RNA, 20 nt, synthetic construct
  source 1..20: mol_type = other RNA
tggagccgaaggtggagttg

SEQ ID NO: 12509 - RNA, 20 nt, synthetic construct
  source 1..20: mol_type = other RNA
ttcggctccaccaacctgac

SEQ ID NO: 12510 - RNA, 20 nt, synthetic construct
  source 1..20: mol_type = other RNA
tcggctccaccaacctgaca

SEQ ID NO: 12511 - RNA, 20 nt, synthetic construct
  source 1..20: mol_type = other RNA
tgtcaggttggtggagccga

SEQ ID NO: 12512 - RNA, 20 nt, synthetic construct
  source 1..20: mol_type = other RNA
gaagagccctgtcaggttgg

SEQ ID NO: 12513 - RNA, 20 nt, synthetic construct
  source 1..20: mol_type = other RNA
aaagaagagccctgtcaggt

SEQ ID NO: 12514 - RNA, 20 nt, synthetic construct
  source 1..20: mol_type = other RNA
gtggaaagaagagccctgtc

SEQ ID NO: 12515 - RNA, 20 nt, synthetic construct
  source 1..20: mol_type = other RNA
ttctttccaccccagctcaa

SEQ ID NO: 12516 - RNA, 20 nt, synthetic construct
  source 1..20: mol_type = other RNA
gctgtgccattgagctgggg

SEQ ID NO: 12517 - RNA, 20 nt, synthetic construct
  source 1..20: mol_type = other RNA
ttggctgtgccattgagctg

SEQ ID NO: 12518 - RNA, 20 nt, synthetic construct
  source 1..20: mol_type = other RNA
attggctgtgccattgagct

SEQ ID NO: 12519 - RNA, 20 nt, synthetic construct
  source 1..20: mol_type = other RNA
cattggctgtgccattgagc

SEQ ID NO: 12520 - RNA, 20 nt, synthetic construct
  source 1..20: mol_type = other RNA
ggcacagccaatgacacagc

SEQ ID NO: 12521 - RNA, 20 nt, synthetic construct
  source 1..20: mol_type = other RNA
ctctgggcctgctgtgtcat

SEQ ID NO: 12522 - RNA, 20 nt, synthetic construct
  source 1..20: mol_type = other RNA
cccagagctgcctgaccctt

SEQ ID NO: 12523 - RNA, 20 nt, synthetic construct
  source 1..20: mol_type = other RNA
ccagagctgcctgacccttt

SEQ ID NO: 12524 - RNA, 20 nt, synthetic construct
  source 1..20: mol_type = other RNA
cagagctgcctgaccctttg

SEQ ID NO: 12525 - RNA, 20 nt, synthetic construct
  source 1..20: mol_type = other RNA
agagctgcctgaccctttgg

SEQ ID NO: 12526 - RNA, 20 nt, synthetic construct
  source 1..20: mol_type = other RNA
gagctgcctgaccctttggg

SEQ ID NO: 12527 - RNA, 20 nt, synthetic construct
  source 1..20: mol_type = other RNA
ccaaagggtcaggcagctct

SEQ ID NO: 12528 - RNA, 20 nt, synthetic construct
  source 1..20: mol_type = other RNA
cccaaagggtcaggcagctc

SEQ ID NO: 12529 - RNA, 20 nt, synthetic construct
  source 1..20: mol_type = other RNA
aacagaccccccaaagggtc

SEQ ID NO: 12530 - RNA, 20 nt, synthetic construct
  source 1..20: mol_type = other RNA
catctaacagaccccccaaa

SEQ ID NO: 12531 - RNA, 20 nt, synthetic construct
  source 1..20: mol_type = other RNA
tcatctaacagaccccccaa

SEQ ID NO: 12532 - RNA, 20 nt, synthetic construct
  source 1..20: mol_type = other RNA
tctgttagatgaagctatgt

SEQ ID NO: 12533 - RNA, 20 nt, synthetic construct
  source 1..20: mol_type = other RNA
gttggatgagatcagcctta

SEQ ID NO: 12534 - RNA, 20 nt, synthetic construct
  source 1..20: mol_type = other RNA
tgagatcagccttatggacc

SEQ ID NO: 12535 - RNA, 20 nt, synthetic construct
  source 1..20: mol_type = other RNA
atggacctggccattgaaga

SEQ ID NO: 12536 - RNA, 20 nt, synthetic construct
  source 1..20: mol_type = other RNA
cttcaatggccaggtccata

SEQ ID NO: 12537 - RNA, 20 nt, synthetic construct
  source 1..20: mol_type = other RNA
taaagccttcttcaatggcc

SEQ ID NO: 12538 - RNA, 20 nt, synthetic construct
  source 1..20: mol_type = other RNA
agggttaaagccttcttcaa

SEQ ID NO: 12539 - RNA, 20 nt, synthetic construct
  source 1..20: mol_type = other RNA
agaaggctttaaccctgtgc

SEQ ID NO: 12540 - RNA, 20 nt, synthetic construct
  source 1..20: mol_type = other RNA
ccctgtgcaggcctcccagc

SEQ ID NO: 12541 - RNA, 20 nt, synthetic construct
  source 1..20: mol_type = other RNA
tgtgcaggcctcccagctgg

SEQ ID NO: 12542 - RNA, 20 nt, synthetic construct
  source 1..20: mol_type = other RNA
ccagctgggaggcctgcaca

SEQ ID NO: 12543 - RNA, 20 nt, synthetic construct
  source 1..20: mol_type = other RNA
gcaggcctcccagctggagg

SEQ ID NO: 12544 - RNA, 20 nt, synthetic construct
  source 1..20: mol_type = other RNA
aaattcctcctccagctggg

SEQ ID NO: 12545 - RNA, 20 nt, synthetic construct
  source 1..20: mol_type = other RNA
gtcaaattcctcctccagct

SEQ ID NO: 12546 - RNA, 20 nt, synthetic construct
  source 1..20: mol_type = other RNA
agtcaaattcctcctccagc

SEQ ID NO: 12547 - RNA, 20 nt, synthetic construct
  source 1..20: mol_type = other RNA
gaggaatttgactctgactc

SEQ ID NO: 12548 - RNA, 20 nt, synthetic construct
  source 1..20: mol_type = other RNA
tatggctcgagtctaaggaa

SEQ ID NO: 12549 - RNA, 20 nt, synthetic construct
  source 1..20: mol_type = other RNA
agggctatggctcgagtcta

SEQ ID NO: 12550 - RNA, 20 nt, synthetic construct
  source 1..20: mol_type = other RNA
tgcttagggaagaagggcta

SEQ ID NO: 12551 - RNA, 20 nt, synthetic construct
  source 1..20: mol_type = other RNA
tcttccctaagcagctctga

SEQ ID NO: 12552 - RNA, 20 nt, synthetic construct
  source 1..20: mol_type = other RNA
cagagctgcttagggaagaa

SEQ ID NO: 12553 - RNA, 20 nt, synthetic construct
  source 1..20: mol_type = other RNA
tcagagctgcttagggaaga

SEQ ID NO: 12554 - RNA, 20 nt, synthetic construct
  source 1..20: mol_type = other RNA
actgccttcagagctgctta

SEQ ID NO: 12555 - RNA, 20 nt, synthetic construct
  source 1..20: mol_type = other RNA
aactgccttcagagctgctt

SEQ ID NO: 12556 - RNA, 20 nt, synthetic construct
  source 1..20: mol_type = other RNA
ggaagaggaggaggaagaag

SEQ ID NO: 12557 - RNA, 20 nt, synthetic construct
  source 1..20: mol_type = other RNA
ggaagaagaggaagaggagg

SEQ ID NO: 12558 - RNA, 20 nt, synthetic construct
  source 1..20: mol_type = other RNA
agaggaagaagaggaagagg

SEQ ID NO: 12559 - RNA, 20 nt, synthetic construct
  source 1..20: mol_type = other RNA
agcagaggaagaagaggaag

SEQ ID NO: 12560 - RNA, 20 nt, synthetic construct
  source 1..20: mol_type = other RNA
ggaagaagcagaggaagaag

SEQ ID NO: 12561 - RNA, 20 nt, synthetic construct
  source 1..20: mol_type = other RNA
agaggcagaggaagaagcag

SEQ ID NO: 12562 - RNA, 20 nt, synthetic construct
  source 1..20: mol_type = other RNA
tgcctcttcctccttttctg

SEQ ID NO: 12563 - RNA, 20 nt, synthetic construct
  source 1..20: mol_type = other RNA
agaaaaggaggaagaggcag

SEQ ID NO: 12564 - RNA, 20 nt, synthetic construct
  source 1..20: mol_type = other RNA
tcttcctccttttctgagga

SEQ ID NO: 12565 - RNA, 20 nt, synthetic construct
  source 1..20: mol_type = other RNA
ttcctcagaaaaggaggaag

SEQ ID NO: 12566 - RNA, 20 nt, synthetic construct
  source 1..20: mol_type = other RNA
ctccttttctgaggaaggtg

SEQ ID NO: 12567 - RNA, 20 nt, synthetic construct
  source 1..20: mol_type = other RNA
cgcaccttcctcagaaaagg

SEQ ID NO: 12568 - RNA, 20 nt, synthetic construct
  source 1..20: mol_type = other RNA
aaccgcaccttcctcagaaa

SEQ ID NO: 12569 - RNA, 20 nt, synthetic construct
  source 1..20: mol_type = other RNA
cagctctgactctgagaccc

SEQ ID NO: 12570 - RNA, 20 nt, synthetic construct
  source 1..20: mol_type = other RNA
tgactctgagaccctggatc

SEQ ID NO: 12571 - RNA, 20 nt, synthetic construct
  source 1..20: mol_type = other RNA
tgagaccctggatctggaag

SEQ ID NO: 12572 - RNA, 20 nt, synthetic construct
  source 1..20: mol_type = other RNA
cctggatctggaagaggccg

SEQ ID NO: 12573 - RNA, 20 nt, synthetic construct
  source 1..20: mol_type = other RNA
ctggatctggaagaggccga

SEQ ID NO: 12574 - RNA, 20 nt, synthetic construct
  source 1..20: mol_type = other RNA
ctcggcctcttccagatcca

SEQ ID NO: 12575 - RNA, 20 nt, synthetic construct
  source 1..20: mol_type = other RNA
cctcggcctcttccagatcc

SEQ ID NO: 12576 - RNA, 20 nt, synthetic construct
  source 1..20: mol_type = other RNA
ggaagaggccgagggtgctg

SEQ ID NO: 12577 - RNA, 20 nt, synthetic construct
  source 1..20: mol_type = other RNA
gaagaggccgagggtgctgt

SEQ ID NO: 12578 - RNA, 20 nt, synthetic construct
  source 1..20: mol_type = other RNA
ctggtagcccacagcaccct

SEQ ID NO: 12579 - RNA, 20 nt, synthetic construct
  source 1..20: mol_type = other RNA
agaacttggaatactcaggc

SEQ ID NO: 12580 - RNA, 20 nt, synthetic construct
  source 1..20: mol_type = other RNA
cggcagaacttggaatactc

SEQ ID NO: 12581 - RNA, 20 nt, synthetic construct
  source 1..20: mol_type = other RNA
gttctgccgcatgagctacc

SEQ ID NO: 12582 - RNA, 20 nt, synthetic construct
  source 1..20: mol_type = other RNA
gtagctcatgcggcagaact

SEQ ID NO: 12583 - RNA, 20 nt, synthetic construct
  source 1..20: mol_type = other RNA
ctggatcctggtagctcatg

SEQ ID NO: 12584 - RNA, 20 nt, synthetic construct
  source 1..20: mol_type = other RNA
atgagagctgagctggatcc

SEQ ID NO: 12585 - RNA, 20 nt, synthetic construct
  source 1..20: mol_type = other RNA
ggcaggcatgagagctgagc

SEQ ID NO: 12586 - RNA, 20 nt, synthetic construct
  source 1..20: mol_type = other RNA
gctctcatgcctgccctacc

SEQ ID NO: 12587 - RNA, 20 nt, synthetic construct
  source 1..20: mol_type = other RNA
cctgccctacctggagcacg

SEQ ID NO: 12588 - RNA, 20 nt, synthetic construct
  source 1..20: mol_type = other RNA
ctgccctacctggagcacgt

SEQ ID NO: 12589 - RNA, 20 nt, synthetic construct
  source 1..20: mol_type = other RNA
ccacgtgctccaggtagggc

SEQ ID NO: 12590 - RNA, 20 nt, synthetic construct
  source 1..20: mol_type = other RNA
tggcccacgtgctccaggta

SEQ ID NO: 12591 - RNA, 20 nt, synthetic construct
  source 1..20: mol_type = other RNA
gtggcccacgtgctccaggt

SEQ ID NO: 12592 - RNA, 20 nt, synthetic construct
  source 1..20: mol_type = other RNA
ggttgtggcccacgtgctcc

SEQ ID NO: 12593 - RNA, 20 nt, synthetic construct
  source 1..20: mol_type = other RNA
ccacaaccacacatacaaca

SEQ ID NO: 12594 - RNA, 20 nt, synthetic construct
  source 1..20: mol_type = other RNA
ccatgttgtatgtgtggttg

SEQ ID NO: 12595 - RNA, 20 nt, synthetic construct
  source 1..20: mol_type = other RNA
tgggtgccatgttgtatgtg

SEQ ID NO: 12596 - RNA, 20 nt, synthetic construct
  source 1..20: mol_type = other RNA
caacatggcacccagtgccc

SEQ ID NO: 12597 - RNA, 20 nt, synthetic construct
  source 1..20: mol_type = other RNA
tcggctgagtccagggcact

SEQ ID NO: 12598 - RNA, 20 nt, synthetic construct
  source 1..20: mol_type = other RNA
gtcggctgagtccagggcac

SEQ ID NO: 12599 - RNA, 20 nt, synthetic construct
  source 1..20: mol_type = other RNA
tggcaggtcggctgagtcca

SEQ ID NO: 12600 - RNA, 20 nt, synthetic construct
  source 1..20: mol_type = other RNA
gtggcaggtcggctgagtcc

SEQ ID NO: 12601 - RNA, 20 nt, synthetic construct
  source 1..20: mol_type = other RNA
ggcactgggtggtggcaggt

SEQ ID NO: 12602 - RNA, 20 nt, synthetic construct
  source 1..20: mol_type = other RNA
tgagggcactgggtggtggc

SEQ ID NO: 12603 - RNA, 20 nt, synthetic construct
  source 1..20: mol_type = other RNA
ccacccagtgccctcaagaa

SEQ ID NO: 12604 - RNA, 20 nt, synthetic construct
  source 1..20: mol_type = other RNA
ttcttgagggcactgggtgg

SEQ ID NO: 12605 - RNA, 20 nt, synthetic construct
  source 1..20: mol_type = other RNA
cctttcttgagggcactggg

SEQ ID NO: 12606 - RNA, 20 nt, synthetic construct
  source 1..20: mol_type = other RNA
tgccctcaagaaaggcagca

SEQ ID NO: 12607 - RNA, 20 nt, synthetic construct
  source 1..20: mol_type = other RNA
gctgcctttcttgagggcac

SEQ ID NO: 12608 - RNA, 20 nt, synthetic construct
  source 1..20: mol_type = other RNA
ctccttgctgcctttcttga

SEQ ID NO: 12609 - RNA, 20 nt, synthetic construct
  source 1..20: mol_type = other RNA
tctccttgctgcctttcttg

SEQ ID NO: 12610 - RNA, 20 nt, synthetic construct
  source 1..20: mol_type = other RNA
gaaaggcagcaaggagaagc

SEQ ID NO: 12611 - RNA, 20 nt, synthetic construct
  source 1..20: mol_type = other RNA
ggagaagcaggctgacttcc

SEQ ID NO: 12612 - RNA, 20 nt, synthetic construct
  source 1..20: mol_type = other RNA
tcctggacaagcagatgagc

SEQ ID NO: 12613 - RNA, 20 nt, synthetic construct
  source 1..20: mol_type = other RNA
cctggacaagcagatgagcc

SEQ ID NO: 12614 - RNA, 20 nt, synthetic construct
  source 1..20: mol_type = other RNA
cccggctcatctgcttgtcc

SEQ ID NO: 12615 - RNA, 20 nt, synthetic construct
  source 1..20: mol_type = other RNA
ctcgggctcggtgctcatcc

SEQ ID NO: 12616 - RNA, 20 nt, synthetic construct
  source 1..20: mol_type = other RNA
ggatcttcatggctcgggct

SEQ ID NO: 12617 - RNA, 20 nt, synthetic construct
  source 1..20: mol_type = other RNA
gaaagggatcttcatggctc

SEQ ID NO: 12618 - RNA, 20 nt, synthetic construct
  source 1..20: mol_type = other RNA
tgaaagggatcttcatggct

SEQ ID NO: 12619 - RNA, 20 nt, synthetic construct
  source 1..20: mol_type = other RNA
attggtgaaagggatcttca

SEQ ID NO: 12620 - RNA, 20 nt, synthetic construct
  source 1..20: mol_type = other RNA
tgattttgtcattggtgaaa

SEQ ID NO: 12621 - RNA, 20 nt, synthetic construct
  source 1..20: mol_type = other RNA
atgattttgtcattggtgaa

SEQ ID NO: 12622 - RNA, 20 nt, synthetic construct
  source 1..20: mol_type = other RNA
caggttgatgattttgtcat

SEQ ID NO: 12623 - RNA, 20 nt, synthetic construct
  source 1..20: mol_type = other RNA
caaaatcatcaacctgcctg

SEQ ID NO: 12624 - RNA, 20 nt, synthetic construct
  source 1..20: mol_type = other RNA
aatcatcaacctgcctgtgg

SEQ ID NO: 12625 - RNA, 20 nt, synthetic construct
  source 1..20: mol_type = other RNA
cattgaactcctccacaggc

SEQ ID NO: 12626 - RNA, 20 nt, synthetic construct
  source 1..20: mol_type = other RNA
agttcattgaactcctccac

SEQ ID NO: 12627 - RNA, 20 nt, synthetic construct
  source 1..20: mol_type = other RNA
ggcttcactcaactggtatt

SEQ ID NO: 12628 - RNA, 20 nt, synthetic construct
  source 1..20: mol_type = other RNA
tcagctgggcttcactcaac

SEQ ID NO: 12629 - RNA, 20 nt, synthetic construct
  source 1..20: mol_type = other RNA
gtctcggatgaggctcagct

SEQ ID NO: 12630 - RNA, 20 nt, synthetic construct
  source 1..20: mol_type = other RNA
tgagcctcatccgagacatc

SEQ ID NO: 12631 - RNA, 20 nt, synthetic construct
  source 1..20: mol_type = other RNA
tcatccgagacatccggcgc

SEQ ID NO: 12632 - RNA, 20 nt, synthetic construct
  source 1..20: mol_type = other RNA
catccgagacatccggcgcc

SEQ ID NO: 12633 - RNA, 20 nt, synthetic construct
  source 1..20: mol_type = other RNA
atccgagacatccggcgccg

SEQ ID NO: 12634 - RNA, 20 nt, synthetic construct
  source 1..20: mol_type = other RNA
ggcgccggatgtctcggatg

SEQ ID NO: 12635 - RNA, 20 nt, synthetic construct
  source 1..20: mol_type = other RNA
tgccccggcgccggatgtct

SEQ ID NO: 12636 - RNA, 20 nt, synthetic construct
  source 1..20: mol_type = other RNA
gcgccggggcaagaacaaga

SEQ ID NO: 12637 - RNA, 20 nt, synthetic construct
  source 1..20: mol_type = other RNA
tcttgttcttgccccggcgc

SEQ ID NO: 12638 - RNA, 20 nt, synthetic construct
  source 1..20: mol_type = other RNA
ccggggcaagaacaagatgg

SEQ ID NO: 12639 - RNA, 20 nt, synthetic construct
  source 1..20: mol_type = other RNA
ccgccatcttgttcttgccc

SEQ ID NO: 12640 - RNA, 20 nt, synthetic construct
  source 1..20: mol_type = other RNA
gaactgccgcaagcgcaagc

SEQ ID NO: 12641 - RNA, 20 nt, synthetic construct
  source 1..20: mol_type = other RNA
tggtgtccagcttgcgcttg

SEQ ID NO: 12642 - RNA, 20 nt, synthetic construct
  source 1..20: mol_type = other RNA
gctggacaccatcctgaatc

SEQ ID NO: 12643 - RNA, 20 nt, synthetic construct
  source 1..20: mol_type = other RNA
cctgaatctggagcgtgatg

SEQ ID NO: 12644 - RNA, 20 nt, synthetic construct
  source 1..20: mol_type = other RNA
atcacgctccagattcagga

SEQ ID NO: 12645 - RNA, 20 nt, synthetic construct
  source 1..20: mol_type = other RNA
gaatctggagcgtgatgtgg

SEQ ID NO: 12646 - RNA, 20 nt, synthetic construct
  source 1..20: mol_type = other RNA
ccacatcacgctccagattc

SEQ ID NO: 12647 - RNA, 20 nt, synthetic construct
  source 1..20: mol_type = other RNA
acctgcagcgtgacaaagcc

SEQ ID NO: 12648 - RNA, 20 nt, synthetic construct
  source 1..20: mol_type = other RNA
gccgggctttgtcacgctgc

SEQ ID NO: 12649 - RNA, 20 nt, synthetic construct
  source 1..20: mol_type = other RNA
gtgacaaagcccggctgctg

SEQ ID NO: 12650 - RNA, 20 nt, synthetic construct
  source 1..20: mol_type = other RNA
tgacaaagcccggctgctgc

SEQ ID NO: 12651 - RNA, 20 nt, synthetic construct
  source 1..20: mol_type = other RNA
ccggctgctgcgggagaaag

SEQ ID NO: 12652 - RNA, 20 nt, synthetic construct
  source 1..20: mol_type = other RNA
cactttctcccgcagcagcc

SEQ ID NO: 12653 - RNA, 20 nt, synthetic construct
  source 1..20: mol_type = other RNA
ccactttctcccgcagcagc

SEQ ID NO: 12654 - RNA, 20 nt, synthetic construct
  source 1..20: mol_type = other RNA
tcatctgtcgcagggagcgc

SEQ ID NO: 12655 - RNA, 20 nt, synthetic construct
  source 1..20: mol_type = other RNA
cctgcgacagatgaagcaga

SEQ ID NO: 12656 - RNA, 20 nt, synthetic construct
  source 1..20: mol_type = other RNA
cttctgcttcatctgtcgca

SEQ ID NO: 12657 - RNA, 20 nt, synthetic construct
  source 1..20: mol_type = other RNA
ccttctgcttcatctgtcgc

SEQ ID NO: 12658 - RNA, 20 nt, synthetic construct
  source 1..20: mol_type = other RNA
gaaggtccagagcctgtacc

SEQ ID NO: 12659 - RNA, 20 nt, synthetic construct
  source 1..20: mol_type = other RNA
ggtccagagcctgtaccagg

SEQ ID NO: 12660 - RNA, 20 nt, synthetic construct
  source 1..20: mol_type = other RNA
agcctgtaccaggaggtgtt

SEQ ID NO: 12661 - RNA, 20 nt, synthetic construct
  source 1..20: mol_type = other RNA
gcctgtaccaggaggtgttt

SEQ ID NO: 12662 - RNA, 20 nt, synthetic construct
  source 1..20: mol_type = other RNA
tgtaccaggaggtgtttggg

SEQ ID NO: 12663 - RNA, 20 nt, synthetic construct
  source 1..20: mol_type = other RNA
gcccaaacacctcctggtac

SEQ ID NO: 12664 - RNA, 20 nt, synthetic construct
  source 1..20: mol_type = other RNA
gcagccgcccaaacacctcc

SEQ ID NO: 12665 - RNA, 20 nt, synthetic construct
  source 1..20: mol_type = other RNA
gggcggctgcgagatgagaa

SEQ ID NO: 12666 - RNA, 20 nt, synthetic construct
  source 1..20: mol_type = other RNA
gcatactgactgggcgagta

SEQ ID NO: 12667 - RNA, 20 nt, synthetic construct
  source 1..20: mol_type = other RNA
cgcatactgactgggcgagt

SEQ ID NO: 12668 - RNA, 20 nt, synthetic construct
  source 1..20: mol_type = other RNA
tactggagcgcatactgact

SEQ ID NO: 12669 - RNA, 20 nt, synthetic construct
  source 1..20: mol_type = other RNA
cagtatgcgctccagtacgc

SEQ ID NO: 12670 - RNA, 20 nt, synthetic construct
  source 1..20: mol_type = other RNA
agtatgcgctccagtacgcc

SEQ ID NO: 12671 - RNA, 20 nt, synthetic construct
  source 1..20: mol_type = other RNA
gtatgcgctccagtacgccg

SEQ ID NO: 12672 - RNA, 20 nt, synthetic construct
  source 1..20: mol_type = other RNA
gcgctccagtacgccgggga

SEQ ID NO: 12673 - RNA, 20 nt, synthetic construct
  source 1..20: mol_type = other RNA
cactgccgtccccggcgtac

SEQ ID NO: 12674 - RNA, 20 nt, synthetic construct
  source 1..20: mol_type = other RNA
gaggaggacactgccgtccc

SEQ ID NO: 12675 - RNA, 20 nt, synthetic construct
  source 1..20: mol_type = other RNA
cctcctcatcccccgcacga

SEQ ID NO: 12676 - RNA, 20 nt, synthetic construct
  source 1..20: mol_type = other RNA
ccatcgtgcgggggatgagg

SEQ ID NO: 12677 - RNA, 20 nt, synthetic construct
  source 1..20: mol_type = other RNA
cggccatcgtgcgggggatg

SEQ ID NO: 12678 - RNA, 20 nt, synthetic construct
  source 1..20: mol_type = other RNA
ccgcacgatggccgaccagc

SEQ ID NO: 12679 - RNA, 20 nt, synthetic construct
  source 1..20: mol_type = other RNA
gctggtcggccatcgtgcgg

SEQ ID NO: 12680 - RNA, 20 nt, synthetic construct
  source 1..20: mol_type = other RNA
tgctggtcggccatcgtgcg

SEQ ID NO: 12681 - RNA, 20 nt, synthetic construct
  source 1..20: mol_type = other RNA
ctgctggtcggccatcgtgc

SEQ ID NO: 12682 - RNA, 20 nt, synthetic construct
  source 1..20: mol_type = other RNA
cgatggccgaccagcaggcc

SEQ ID NO: 12683 - RNA, 20 nt, synthetic construct
  source 1..20: mol_type = other RNA
tggccgaccagcaggcccgg

SEQ ID NO: 12684 - RNA, 20 nt, synthetic construct
  source 1..20: mol_type = other RNA
cgaccagcaggcccggcggc

SEQ ID NO: 12685 - RNA, 20 nt, synthetic construct
  source 1..20: mol_type = other RNA
ctgccgccgggcctgctggt

SEQ ID NO: 12686 - RNA, 20 nt, synthetic construct
  source 1..20: mol_type = other RNA
agcaggcccggcggcaggag

SEQ ID NO: 12687 - RNA, 20 nt, synthetic construct
  source 1..20: mol_type = other RNA
tctcctgccgccgggcctgc

SEQ ID NO: 12688 - RNA, 20 nt, synthetic construct
  source 1..20: mol_type = other RNA
gcggcaggagaggaagccaa

SEQ ID NO: 12689 - RNA, 20 nt, synthetic construct
  source 1..20: mol_type = other RNA
tggcttcctctcctgccgcc

SEQ ID NO: 12690 - RNA, 20 nt, synthetic construct
  source 1..20: mol_type = other RNA
ttggcttcctctcctgccgc

SEQ ID NO: 12691 - RNA, 20 nt, synthetic construct
  source 1..20: mol_type = other RNA
aggagaggaagccaaaggac

SEQ ID NO: 12692 - RNA, 20 nt, synthetic construct
  source 1..20: mol_type = other RNA
aggaccggagaaagtgagcc

SEQ ID NO: 12693 - RNA, 20 nt, synthetic construct
  source 1..20: mol_type = other RNA
gctcactttctccggtcctt

SEQ ID NO: 12694 - RNA, 20 nt, synthetic construct
  source 1..20: mol_type = other RNA
gaccggagaaagtgagcctg

SEQ ID NO: 12695 - RNA, 20 nt, synthetic construct
  source 1..20: mol_type = other RNA
gaaagtgagcctggggaaga

SEQ ID NO: 12696 - RNA, 20 nt, synthetic construct
  source 1..20: mol_type = other RNA
aaagtgagcctggggaagaa

SEQ ID NO: 12697 - RNA, 20 nt, synthetic construct
  source 1..20: mol_type = other RNA
aagtgagcctggggaagaag

SEQ ID NO: 12698 - RNA, 20 nt, synthetic construct
  source 1..20: mol_type = other RNA
agtgagcctggggaagaagg

SEQ ID NO: 12699 - RNA, 20 nt, synthetic construct
  source 1..20: mol_type = other RNA
ttcaaacccccttcttcccc

SEQ ID NO: 12700 - RNA, 20 nt, synthetic construct
  source 1..20: mol_type = other RNA
aagcccaccaagaccgaaac

SEQ ID NO: 12701 - RNA, 20 nt, synthetic construct
  source 1..20: mol_type = other RNA
accaagaccgaaactggaga

SEQ ID NO: 12702 - RNA, 20 nt, synthetic construct
  source 1..20: mol_type = other RNA
ccaagaccgaaactggagaa

SEQ ID NO: 12703 - RNA, 20 nt, synthetic construct
  source 1..20: mol_type = other RNA
tctccagtttcggtcttggt

SEQ ID NO: 12704 - RNA, 20 nt, synthetic construct
  source 1..20: mol_type = other RNA
ttctccagtttcggtcttgg

SEQ ID NO: 12705 - RNA, 20 nt, synthetic construct
  source 1..20: mol_type = other RNA
gaccgaaactggagaagggc

SEQ ID NO: 12706 - RNA, 20 nt, synthetic construct
  source 1..20: mol_type = other RNA
cccttctccagtttcggtct

SEQ ID NO: 12707 - RNA, 20 nt, synthetic construct
  source 1..20: mol_type = other RNA
aactggagaagggctggacc

SEQ ID NO: 12708 - RNA, 20 nt, synthetic construct
  source 1..20: mol_type = other RNA
gtccagcccttctccagttt

SEQ ID NO: 12709 - RNA, 20 nt, synthetic construct
  source 1..20: mol_type = other RNA
agaagggctggacctggacc

SEQ ID NO: 12710 - RNA, 20 nt, synthetic construct
  source 1..20: mol_type = other RNA
gctggacctggacctggacc

SEQ ID NO: 12711 - RNA, 20 nt, synthetic construct
  source 1..20: mol_type = other RNA
acctggacctggacctacag

SEQ ID NO: 12712 - RNA, 20 nt, synthetic construct
  source 1..20: mol_type = other RNA
cctggacctggacctacagc

SEQ ID NO: 12713 - RNA, 20 nt, synthetic construct
  source 1..20: mol_type = other RNA
ctggacctggacctacagcg

SEQ ID NO: 12714 - RNA, 20 nt, synthetic construct
  source 1..20: mol_type = other RNA
cccgctgtaggtccaggtcc

SEQ ID NO: 12715 - RNA, 20 nt, synthetic construct
  source 1..20: mol_type = other RNA
taagtccccgctgtaggtcc

SEQ ID NO: 12716 - RNA, 20 nt, synthetic construct
  source 1..20: mol_type = other RNA
ggcatttaagtccccgctgt

SEQ ID NO: 12717 - RNA, 20 nt, synthetic construct
  source 1..20: mol_type = other RNA
agaagatatattggataaga

SEQ ID NO: 12718 - RNA, 20 nt, synthetic construct
  source 1..20: mol_type = other RNA
atccaatatatcttctcaga

SEQ ID NO: 12719 - RNA, 20 nt, synthetic construct
  source 1..20: mol_type = other RNA
tccaatatatcttctcagat

SEQ ID NO: 12720 - RNA, 20 nt, synthetic construct
  source 1..20: mol_type = other RNA
tcccatctgagaagatatat

SEQ ID NO: 12721 - RNA, 20 nt, synthetic construct
  source 1..20: mol_type = other RNA
cttctcagatgggatgactg

SEQ ID NO: 12722 - RNA, 20 nt, synthetic construct
  source 1..20: mol_type = other RNA
ttctcagatgggatgactgc

SEQ ID NO: 12723 - RNA, 20 nt, synthetic construct
  source 1..20: mol_type = other RNA
atgactgcgggtcagtgtac

SEQ ID NO: 12724 - RNA, 20 nt, synthetic construct
  source 1..20: mol_type = other RNA
gcgggtcagtgtacaggaag

SEQ ID NO: 12725 - RNA, 20 nt, synthetic construct
  source 1..20: mol_type = other RNA
gtcagtgtacaggaagaggc

SEQ ID NO: 12726 - RNA, 20 nt, synthetic construct
  source 1..20: mol_type = other RNA
gtacaggaagaggcaggcac

SEQ ID NO: 12727 - RNA, 20 nt, synthetic construct
  source 1..20: mol_type = other RNA
aggaagaggcaggcactggc

SEQ ID NO: 12728 - RNA, 20 nt, synthetic construct
  source 1..20: mol_type = other RNA
ctggctggctcagctccact

SEQ ID NO: 12729 - RNA, 20 nt, synthetic construct
  source 1..20: mol_type = other RNA
tggctggctcagctccactc

SEQ ID NO: 12730 - RNA, 20 nt, synthetic construct
  source 1..20: mol_type = other RNA
ctggctcagctccactcggg

SEQ ID NO: 12731 - RNA, 20 nt, synthetic construct
  source 1..20: mol_type = other RNA
tcagctccactcgggtggag

SEQ ID NO: 12732 - RNA, 20 nt, synthetic construct
  source 1..20: mol_type = other RNA
ccactcgggtggagtggaag

SEQ ID NO: 12733 - RNA, 20 nt, synthetic construct
  source 1..20: mol_type = other RNA
ccacttccactccacccgag

SEQ ID NO: 12734 - RNA, 20 nt, synthetic construct
  source 1..20: mol_type = other RNA
aagtggccagaccatttaga

SEQ ID NO: 12735 - RNA, 20 nt, synthetic construct
  source 1..20: mol_type = other RNA
gccagaccatttagacggac

SEQ ID NO: 12736 - RNA, 20 nt, synthetic construct
  source 1..20: mol_type = other RNA
ccagaccatttagacggaca

SEQ ID NO: 12737 - RNA, 20 nt, synthetic construct
  source 1..20: mol_type = other RNA
ccctgtccgtctaaatggtc

SEQ ID NO: 12738 - RNA, 20 nt, synthetic construct
  source 1..20: mol_type = other RNA
gaggaccctgtccgtctaaa

SEQ ID NO: 12739 - RNA, 20 nt, synthetic construct
  source 1..20: mol_type = other RNA
caccctacccctttcctgtg

SEQ ID NO: 12740 - RNA, 20 nt, synthetic construct
  source 1..20: mol_type = other RNA
cacaggaaaggggtagggtg

SEQ ID NO: 12741 - RNA, 20 nt, synthetic construct
  source 1..20: mol_type = other RNA
ctacccctttcctgtgaggc

SEQ ID NO: 12742 - RNA, 20 nt, synthetic construct
  source 1..20: mol_type = other RNA
tacccctttcctgtgaggca

SEQ ID NO: 12743 - RNA, 20 nt, synthetic construct
  source 1..20: mol_type = other RNA
acccctttcctgtgaggcag

SEQ ID NO: 12744 - RNA, 20 nt, synthetic construct
  source 1..20: mol_type = other RNA
tgcctcacaggaaaggggta

SEQ ID NO: 12745 - RNA, 20 nt, synthetic construct
  source 1..20: mol_type = other RNA
ctgcctcacaggaaaggggt

SEQ ID NO: 12746 - RNA, 20 nt, synthetic construct
  source 1..20: mol_type = other RNA
cctttcctgtgaggcagggg

SEQ ID NO: 12747 - RNA, 20 nt, synthetic construct
  source 1..20: mol_type = other RNA
acccctgcctcacaggaaag

SEQ ID NO: 12748 - RNA, 20 nt, synthetic construct
  source 1..20: mol_type = other RNA
cacccctgcctcacaggaaa

SEQ ID NO: 12749 - RNA, 20 nt, synthetic construct
  source 1..20: mol_type = other RNA
ccacccctgcctcacaggaa

SEQ ID NO: 12750 - RNA, 20 nt, synthetic construct
  source 1..20: mol_type = other RNA
ctgtgaggcaggggtggtgg

SEQ ID NO: 12751 - RNA, 20 nt, synthetic construct
  source 1..20: mol_type = other RNA
caccaccacccctgcctcac

SEQ ID NO: 12752 - RNA, 20 nt, synthetic construct
  source 1..20: mol_type = other RNA
aggggtggtggtggagttgc

SEQ ID NO: 12753 - RNA, 20 nt, synthetic construct
  source 1..20: mol_type = other RNA
ggtggtggtggagttgctgg

SEQ ID NO: 12754 - RNA, 20 nt, synthetic construct
  source 1..20: mol_type = other RNA
ggtggagttgctggaggtag

SEQ ID NO: 12755 - RNA, 20 nt, synthetic construct
  source 1..20: mol_type = other RNA
ctggaggtagaggagctatg

SEQ ID NO: 12756 - RNA, 20 nt, synthetic construct
  source 1..20: mol_type = other RNA
agaggagctatgtggagcaa

SEQ ID NO: 12757 - RNA, 20 nt, synthetic construct
  source 1..20: mol_type = other RNA
tgtggagcaaaggccgacag

SEQ ID NO: 12758 - RNA, 20 nt, synthetic construct
  source 1..20: mol_type = other RNA
gtggagcaaaggccgacaga

SEQ ID NO: 12759 - RNA, 20 nt, synthetic construct
  source 1..20: mol_type = other RNA
tggagcaaaggccgacagag

SEQ ID NO: 12760 - RNA, 20 nt, synthetic construct
  source 1..20: mol_type = other RNA
gcaaaggccgacagagggga

SEQ ID NO: 12761 - RNA, 20 nt, synthetic construct
  source 1..20: mol_type = other RNA
ggccgacagaggggaaggaa

SEQ ID NO: 12762 - RNA, 20 nt, synthetic construct
  source 1..20: mol_type = other RNA
gtccattccttcccctctgt

SEQ ID NO: 12763 - RNA, 20 nt, synthetic construct
  source 1..20: mol_type = other RNA
ggaaggaatggacctgtgag

SEQ ID NO: 12764 - RNA, 20 nt, synthetic construct
  source 1..20: mol_type = other RNA
ggaatggacctgtgagagga

SEQ ID NO: 12765 - RNA, 20 nt, synthetic construct
  source 1..20: mol_type = other RNA
gaatggacctgtgagaggaa

SEQ ID NO: 12766 - RNA, 20 nt, synthetic construct
  source 1..20: mol_type = other RNA
ggacctgtgagaggaaggga

SEQ ID NO: 12767 - RNA, 20 nt, synthetic construct
  source 1..20: mol_type = other RNA
cctgtgagaggaagggaagg

SEQ ID NO: 12768 - RNA, 20 nt, synthetic construct
  source 1..20: mol_type = other RNA
ccaccttcccttcctctcac

SEQ ID NO: 12769 - RNA, 20 nt, synthetic construct
  source 1..20: mol_type = other RNA
gtggcagaaagtctcatttc

SEQ ID NO: 12770 - RNA, 20 nt, synthetic construct
  source 1..20: mol_type = other RNA
cagaaagtctcatttcagga

SEQ ID NO: 12771 - RNA, 20 nt, synthetic construct
  source 1..20: mol_type = other RNA
aaagtctcatttcaggaagg

SEQ ID NO: 12772 - RNA, 20 nt, synthetic construct
  source 1..20: mol_type = other RNA
aagtctcatttcaggaagga

SEQ ID NO: 12773 - RNA, 20 nt, synthetic construct
  source 1..20: mol_type = other RNA
tttcaggaaggagggataga

SEQ ID NO: 12774 - RNA, 20 nt, synthetic construct
  source 1..20: mol_type = other RNA
aggaaggagggatagaagga

SEQ ID NO: 12775 - RNA, 20 nt, synthetic construct
  source 1..20: mol_type = other RNA
aggagggatagaaggaagga

SEQ ID NO: 12776 - RNA, 20 nt, synthetic construct
  source 1..20: mol_type = other RNA
gggatagaaggaaggaagga

SEQ ID NO: 12777 - RNA, 20 nt, synthetic construct
  source 1..20: mol_type = other RNA
tttttttttcgggggggggg

SEQ ID NO: 12778 - RNA, 20 nt, synthetic construct
  source 1..20: mol_type = other RNA
atttttttttcggggggggg

SEQ ID NO: 12779 - RNA, 20 nt, synthetic construct
  source 1..20: mol_type = other RNA
gatttttttttcgggggggg

SEQ ID NO: 12780 - RNA, 20 nt, synthetic construct
  source 1..20: mol_type = other RNA
tgatttttttttcggggggg

SEQ ID NO: 12781 - RNA, 20 nt, synthetic construct
  source 1..20: mol_type = other RNA
ttgatttttttttcgggggg

SEQ ID NO: 12782 - RNA, 20 nt, synthetic construct
  source 1..20: mol_type = other RNA
cccgaaaaaaaaatcaaagc

SEQ ID NO: 12783 - RNA, 20 nt, synthetic construct
  source 1..20: mol_type = other RNA
ctttgatttttttttcgggg

SEQ ID NO: 12784 - RNA, 20 nt, synthetic construct
  source 1..20: mol_type = other RNA
gctttgatttttttttcggg

SEQ ID NO: 12785 - RNA, 20 nt, synthetic construct
  source 1..20: mol_type = other RNA
cgctttgatttttttttcgg

SEQ ID NO: 12786 - RNA, 20 nt, synthetic construct
  source 1..20: mol_type = other RNA
ccgctttgatttttttttcg

SEQ ID NO: 12787 - RNA, 20 nt, synthetic construct
  source 1..20: mol_type = other RNA
cccgctttgatttttttttc

SEQ ID NO: 12788 - RNA, 20 nt, synthetic construct
  source 1..20: mol_type = other RNA
tcccgctttgattttttttt

SEQ ID NO: 12789 - RNA, 20 nt, synthetic construct
  source 1..20: mol_type = other RNA
caaagcgggaagaaaatcag

SEQ ID NO: 12790 - RNA, 20 nt, synthetic construct
  source 1..20: mol_type = other RNA
aaagcgggaagaaaatcaga

SEQ ID NO: 12791 - RNA, 20 nt, synthetic construct
  source 1..20: mol_type = other RNA
cgggaagaaaatcagaggga

SEQ ID NO: 12792 - RNA, 20 nt, synthetic construct
  source 1..20: mol_type = other RNA
gaaaatcagagggaaggtta

SEQ ID NO: 12793 - RNA, 20 nt, synthetic construct
  source 1..20: mol_type = other RNA
atcagagggaaggttaaggt

SEQ ID NO: 12794 - RNA, 20 nt, synthetic construct
  source 1..20: mol_type = other RNA
gggaaggttaaggttggctc

SEQ ID NO: 12795 - RNA, 20 nt, synthetic construct
  source 1..20: mol_type = other RNA
ggttaaggttggctctggcc

SEQ ID NO: 12796 - RNA, 20 nt, synthetic construct
  source 1..20: mol_type = other RNA
ttggctctggccaggattcc

SEQ ID NO: 12797 - RNA, 20 nt, synthetic construct
  source 1..20: mol_type = other RNA
tggccaggattccaggcagc

SEQ ID NO: 12798 - RNA, 20 nt, synthetic construct
  source 1..20: mol_type = other RNA
caggattccaggcagcaggt

SEQ ID NO: 12799 - RNA, 20 nt, synthetic construct
  source 1..20: mol_type = other RNA
caacctgctgcctggaatcc

SEQ ID NO: 12800 - RNA, 20 nt, synthetic construct
  source 1..20: mol_type = other RNA
aggcagcaggttggagtgac

SEQ ID NO: 12801 - RNA, 20 nt, synthetic construct
  source 1..20: mol_type = other RNA
agtcactccaacctgctgcc

SEQ ID NO: 12802 - RNA, 20 nt, synthetic construct
  source 1..20: mol_type = other RNA
agcaggttggagtgactggt

SEQ ID NO: 12803 - RNA, 20 nt, synthetic construct
  source 1..20: mol_type = other RNA
gactggtgggcctagatcac

SEQ ID NO: 12804 - RNA, 20 nt, synthetic construct
  source 1..20: mol_type = other RNA
gtttatcacaccagtgatct

SEQ ID NO: 12805 - RNA, 20 nt, synthetic construct
  source 1..20: mol_type = other RNA
ataaaccccaattttcaccc

SEQ ID NO: 12806 - RNA, 20 nt, synthetic construct
  source 1..20: mol_type = other RNA
taaaccccaattttcacccc

SEQ ID NO: 12807 - RNA, 20 nt, synthetic construct
  source 1..20: mol_type = other RNA
aaaccccaattttcaccccg

SEQ ID NO: 12808 - RNA, 20 nt, synthetic construct
  source 1..20: mol_type = other RNA
aaccccaattttcaccccgg

SEQ ID NO: 12809 - RNA, 20 nt, synthetic construct
  source 1..20: mol_type = other RNA
accccaattttcaccccggg

SEQ ID NO: 12810 - RNA, 20 nt, synthetic construct
  source 1..20: mol_type = other RNA
ccccaattttcaccccgggg

SEQ ID NO: 12811 - RNA, 20 nt, synthetic construct
  source 1..20: mol_type = other RNA
cccaattttcaccccggggg

SEQ ID NO: 12812 - RNA, 20 nt, synthetic construct
  source 1..20: mol_type = other RNA
aattttcaccccgggggggg

SEQ ID NO: 12813 - RNA, 20 nt, synthetic construct
  source 1..20: mol_type = other RNA
cccccccggggtgaaaattg

SEQ ID NO: 12814 - RNA, 20 nt, synthetic construct
  source 1..20: mol_type = other RNA
ccccccccggggtgaaaatt

SEQ ID NO: 12815 - RNA, 20 nt, synthetic construct
  source 1..20: mol_type = other RNA
accccccccggggtgaaaat

SEQ ID NO: 12816 - RNA, 20 nt, synthetic construct
  source 1..20: mol_type = other RNA
tgtgtaccccaccccccccg

SEQ ID NO: 12817 - RNA, 20 nt, synthetic construct
  source 1..20: mol_type = other RNA
ctgtgtaccccacccccccc

SEQ ID NO: 12818 - RNA, 20 nt, synthetic construct
  source 1..20: mol_type = other RNA
tctgtgtaccccaccccccc

SEQ ID NO: 12819 - RNA, 20 nt, synthetic construct
  source 1..20: mol_type = other RNA
ggggtggggtacacagacac

SEQ ID NO: 12820 - RNA, 20 nt, synthetic construct
  source 1..20: mol_type = other RNA
gggtggggtacacagacaca

SEQ ID NO: 12821 - RNA, 20 nt, synthetic construct
  source 1..20: mol_type = other RNA
tggggtacacagacacaggg

SEQ ID NO: 12822 - RNA, 20 nt, synthetic construct
  source 1..20: mol_type = other RNA
ggggtacacagacacagggt

SEQ ID NO: 12823 - RNA, 20 nt, synthetic construct
  source 1..20: mol_type = other RNA
gggtacacagacacagggtg

SEQ ID NO: 12824 - RNA, 20 nt, synthetic construct
  source 1..20: mol_type = other RNA
ggtacacagacacagggtgg

SEQ ID NO: 12825 - RNA, 20 nt, synthetic construct
  source 1..20: mol_type = other RNA
acacagacacagggtggggg

SEQ ID NO: 12826 - RNA, 20 nt, synthetic construct
  source 1..20: mol_type = other RNA
cacagacacagggtgggggt

SEQ ID NO: 12827 - RNA, 20 nt, synthetic construct
  source 1..20: mol_type = other RNA
acagacacagggtgggggtg

SEQ ID NO: 12828 - RNA, 20 nt, synthetic construct
  source 1..20: mol_type = other RNA
gacacagggtgggggtgggg

SEQ ID NO: 12829 - RNA, 20 nt, synthetic construct
  source 1..20: mol_type = other RNA
acacagggtgggggtgggga

SEQ ID NO: 12830 - RNA, 20 nt, synthetic construct
  source 1..20: mol_type = other RNA
agggtgggggtggggaggga

SEQ ID NO: 12831 - RNA, 20 nt, synthetic construct
  source 1..20: mol_type = other RNA
ttgcattttgacatccctga

SEQ ID NO: 12832 - RNA, 20 nt, synthetic construct
  source 1..20: mol_type = other RNA
tgcattttgacatccctgaa

SEQ ID NO: 12833 - RNA, 20 nt, synthetic construct
  source 1..20: mol_type = other RNA
gcattttgacatccctgaag

SEQ ID NO: 12834 - RNA, 20 nt, synthetic construct
  source 1..20: mol_type = other RNA
ttcagggatgtcaaaatgca

SEQ ID NO: 12835 - RNA, 20 nt, synthetic construct
  source 1..20: mol_type = other RNA
catccctgaaggggagctct

SEQ ID NO: 12836 - RNA, 20 nt, synthetic construct
  source 1..20: mol_type = other RNA
tatccaagagctccccttca

SEQ ID NO: 12837 - RNA, 20 nt, synthetic construct
  source 1..20: mol_type = other RNA
atatccaagagctccccttc

SEQ ID NO: 12838 - RNA, 20 nt, synthetic construct
  source 1..20: mol_type = other RNA
ggggagctcttggatatcat

SEQ ID NO: 12839 - RNA, 20 nt, synthetic construct
  source 1..20: mol_type = other RNA
ttggccatgtttcaatcgaa

SEQ ID NO: 12840 - RNA, 20 nt, synthetic construct
  source 1..20: mol_type = other RNA
tttcaatcgaatggagccac

SEQ ID NO: 12841 - RNA, 20 nt, synthetic construct
  source 1..20: mol_type = other RNA
ttcaatcgaatggagccact

SEQ ID NO: 12842 - RNA, 20 nt, synthetic construct
  source 1..20: mol_type = other RNA
gagccactgggccccaacac

SEQ ID NO: 12843 - RNA, 20 nt, synthetic construct
  source 1..20: mol_type = other RNA
aagccagtgttggggcccag

SEQ ID NO: 12844 - RNA, 20 nt, synthetic construct
  source 1..20: mol_type = other RNA
aaatctcaaagccagtgttg

SEQ ID NO: 12845 - RNA, 20 nt, synthetic construct
  source 1..20: mol_type = other RNA
taaatctcaaagccagtgtt

SEQ ID NO: 12846 - RNA, 20 nt, synthetic construct
  source 1..20: mol_type = other RNA
ctaaatctcaaagccagtgt

SEQ ID NO: 12847 - RNA, 20 nt, synthetic construct
  source 1..20: mol_type = other RNA
gctttgagatttagagtcaa

SEQ ID NO: 12848 - RNA, 20 nt, synthetic construct
  source 1..20: mol_type = other RNA
ctttgagatttagagtcaaa

SEQ ID NO: 12849 - RNA, 20 nt, synthetic construct
  source 1..20: mol_type = other RNA
agtcaaagggtagagtgaac

SEQ ID NO: 12850 - RNA, 20 nt, synthetic construct
  source 1..20: mol_type = other RNA
aagggtagagtgaacaggaa

SEQ ID NO: 12851 - RNA, 20 nt, synthetic construct
  source 1..20: mol_type = other RNA
agggtagagtgaacaggaaa

SEQ ID NO: 12852 - RNA, 20 nt, synthetic construct
  source 1..20: mol_type = other RNA
gtgaacaggaaagggtcacg

SEQ ID NO: 12853 - RNA, 20 nt, synthetic construct
  source 1..20: mol_type = other RNA
tgttggggctgttgcaacat

SEQ ID NO: 12854 - RNA, 20 nt, synthetic construct
  source 1..20: mol_type = other RNA
atgttggggctgttgcaaca

SEQ ID NO: 12855 - RNA, 20 nt, synthetic construct
  source 1..20: mol_type = other RNA
gaatgacatgcgtgatgttg

SEQ ID NO: 12856 - RNA, 20 nt, synthetic construct
  source 1..20: mol_type = other RNA
tgaatgacatgcgtgatgtt

SEQ ID NO: 12857 - RNA, 20 nt, synthetic construct
  source 1..20: mol_type = other RNA
gtgaatgacatgcgtgatgt

SEQ ID NO: 12858 - RNA, 20 nt, synthetic construct
  source 1..20: mol_type = other RNA
cggagggagatggagtggca

SEQ ID NO: 12859 - RNA, 20 nt, synthetic construct
  source 1..20: mol_type = other RNA
gagcacggagggagatggag

SEQ ID NO: 12860 - RNA, 20 nt, synthetic construct
  source 1..20: mol_type = other RNA
ggctggagcacggagggaga

SEQ ID NO: 12861 - RNA, 20 nt, synthetic construct
  source 1..20: mol_type = other RNA
aggggtggctggagcacgga

SEQ ID NO: 12862 - RNA, 20 nt, synthetic construct
  source 1..20: mol_type = other RNA
caggggtggctggagcacgg

SEQ ID NO: 12863 - RNA, 20 nt, synthetic construct
  source 1..20: mol_type = other RNA
ctccagccacccctgagctg

SEQ ID NO: 12864 - RNA, 20 nt, synthetic construct
  source 1..20: mol_type = other RNA
agcctcagctcaggggtggc

SEQ ID NO: 12865 - RNA, 20 nt, synthetic construct
  source 1..20: mol_type = other RNA
tgggagcctcagctcagggg

SEQ ID NO: 12866 - RNA, 20 nt, synthetic construct
  source 1..20: mol_type = other RNA
caatgggagcctcagctcag

SEQ ID NO: 12867 - RNA, 20 nt, synthetic construct
  source 1..20: mol_type = other RNA
acaatgggagcctcagctca

SEQ ID NO: 12868 - RNA, 20 nt, synthetic construct
  source 1..20: mol_type = other RNA
gacaatgggagcctcagctc

SEQ ID NO: 12869 - RNA, 20 nt, synthetic construct
  source 1..20: mol_type = other RNA
caggctctgatggagacaat

SEQ ID NO: 12870 - RNA, 20 nt, synthetic construct
  source 1..20: mol_type = other RNA
gcaggctctgatggagacaa

SEQ ID NO: 12871 - RNA, 20 nt, synthetic construct
  source 1..20: mol_type = other RNA
catacacatgcaggctctga

SEQ ID NO: 12872 - RNA, 20 nt, synthetic construct
  source 1..20: mol_type = other RNA
atgtgtatgccgtcctcccc

SEQ ID NO: 12873 - RNA, 20 nt, synthetic construct
  source 1..20: mol_type = other RNA
tatgccgtcctcccctggtc

SEQ ID NO: 12874 - RNA, 20 nt, synthetic construct
  source 1..20: mol_type = other RNA
aacaccggaccaggggagga

SEQ ID NO: 12875 - RNA, 20 nt, synthetic construct
  source 1..20: mol_type = other RNA
cacaaacaccggaccagggg

SEQ ID NO: 12876 - RNA, 20 nt, synthetic construct
  source 1..20: mol_type = other RNA
gaacacaaacaccggaccag

SEQ ID NO: 12877 - RNA, 20 nt, synthetic construct
  source 1..20: mol_type = other RNA
ggaacacaaacaccggacca

SEQ ID NO: 12878 - RNA, 20 nt, synthetic construct
  source 1..20: mol_type = other RNA
gggaacacaaacaccggacc

SEQ ID NO: 12879 - RNA, 20 nt, synthetic construct
  source 1..20: mol_type = other RNA
ggggtggggaacacaaacac

SEQ ID NO: 12880 - RNA, 20 nt, synthetic construct
  source 1..20: mol_type = other RNA
caggcagtctgtgaggggtg

SEQ ID NO: 12881 - RNA, 20 nt, synthetic construct
  source 1..20: mol_type = other RNA
tcaggcagtctgtgaggggt

SEQ ID NO: 12882 - RNA, 20 nt, synthetic construct
  source 1..20: mol_type = other RNA
ctcaggcagtctgtgagggg

SEQ ID NO: 12883 - RNA, 20 nt, synthetic construct
  source 1..20: mol_type = other RNA
gagctcaggcagtctgtgag

SEQ ID NO: 12884 - RNA, 20 nt, synthetic construct
  source 1..20: mol_type = other RNA
agagctcaggcagtctgtga

SEQ ID NO: 12885 - RNA, 20 nt, synthetic construct
  source 1..20: mol_type = other RNA
aagagctcaggcagtctgtg

SEQ ID NO: 12886 - RNA, 20 nt, synthetic construct
  source 1..20: mol_type = other RNA
gcctgagctcttctgtaagc

SEQ ID NO: 12887 - RNA, 20 nt, synthetic construct
  source 1..20: mol_type = other RNA
cctgagctcttctgtaagct

SEQ ID NO: 12888 - RNA, 20 nt, synthetic construct
  source 1..20: mol_type = other RNA
ctgagctcttctgtaagctg

SEQ ID NO: 12889 - RNA, 20 nt, synthetic construct
  source 1..20: mol_type = other RNA
cccagcttacagaagagctc

SEQ ID NO: 12890 - RNA, 20 nt, synthetic construct
  source 1..20: mol_type = other RNA
ctcttctgtaagctggggta

SEQ ID NO: 12891 - RNA, 20 nt, synthetic construct
  source 1..20: mol_type = other RNA
tgtaagctggggtagggtga

SEQ ID NO: 12892 - RNA, 20 nt, synthetic construct
  source 1..20: mol_type = other RNA
gtagggtgatggcagtgctc

SEQ ID NO: 12893 - RNA, 20 nt, synthetic construct
  source 1..20: mol_type = other RNA
tagggtgatggcagtgctcc

SEQ ID NO: 12894 - RNA, 20 nt, synthetic construct
  source 1..20: mol_type = other RNA
gatggcagtgctccgggaac

SEQ ID NO: 12895 - RNA, 20 nt, synthetic construct
  source 1..20: mol_type = other RNA
atggcagtgctccgggaact

SEQ ID NO: 12896 - RNA, 20 nt, synthetic construct
  source 1..20: mol_type = other RNA
aaggctgcaggcccagttcc

SEQ ID NO: 12897 - RNA, 20 nt, synthetic construct
  source 1..20: mol_type = other RNA
ggcctgcagccttcctcttc

SEQ ID NO: 12898 - RNA, 20 nt, synthetic construct
  source 1..20: mol_type = other RNA
gcctgcagccttcctcttct

SEQ ID NO: 12899 - RNA, 20 nt, synthetic construct
  source 1..20: mol_type = other RNA
tcccagaagaggaaggctgc

SEQ ID NO: 12900 - RNA, 20 nt, synthetic construct
  source 1..20: mol_type = other RNA
cctcttctgggactgctgtg

SEQ ID NO: 12901 - RNA, 20 nt, synthetic construct
  source 1..20: mol_type = other RNA
acagcagtcccagaagagga

SEQ ID NO: 12902 - RNA, 20 nt, synthetic construct
  source 1..20: mol_type = other RNA
cctcacagcagtcccagaag

SEQ ID NO: 12903 - RNA, 20 nt, synthetic construct
  source 1..20: mol_type = other RNA
ctgggactgctgtgaggcag

SEQ ID NO: 12904 - RNA, 20 nt, synthetic construct
  source 1..20: mol_type = other RNA
gctgtgaggcagaggaatga

SEQ ID NO: 12905 - RNA, 20 nt, synthetic construct
  source 1..20: mol_type = other RNA
aatctagtgtagcagcctcc

SEQ ID NO: 12906 - RNA, 20 nt, synthetic construct
  source 1..20: mol_type = other RNA
tagtgtagcagcctccaggc

SEQ ID NO: 12907 - RNA, 20 nt, synthetic construct
  source 1..20: mol_type = other RNA
ttgtgctgaatcctgcctgg

SEQ ID NO: 12908 - RNA, 20 nt, synthetic construct
  source 1..20: mol_type = other RNA
ggcaggattcagcacaacac

SEQ ID NO: 12909 - RNA, 20 nt, synthetic construct
  source 1..20: mol_type = other RNA
gcaggattcagcacaacact

SEQ ID NO: 12910 - RNA, 20 nt, synthetic construct
  source 1..20: mol_type = other RNA
caggattcagcacaacactg

SEQ ID NO: 12911 - RNA, 20 nt, synthetic construct
  source 1..20: mol_type = other RNA
ctggggagtcacccttccct

SEQ ID NO: 12912 - RNA, 20 nt, synthetic construct
  source 1..20: mol_type = other RNA
tggggagtcacccttccctc

SEQ ID NO: 12913 - RNA, 20 nt, synthetic construct
  source 1..20: mol_type = other RNA
taggcagaggcccgagggaa

SEQ ID NO: 12914 - RNA, 20 nt, synthetic construct
  source 1..20: mol_type = other RNA
gtaggcagaggcccgaggga

SEQ ID NO: 12915 - RNA, 20 nt, synthetic construct
  source 1..20: mol_type = other RNA
gttggtaggcagaggcccga

SEQ ID NO: 12916 - RNA, 20 nt, synthetic construct
  source 1..20: mol_type = other RNA
tgttggtaggcagaggcccg

SEQ ID NO: 12917 - RNA, 20 nt, synthetic construct
  source 1..20: mol_type = other RNA
gcctctgcctaccaacaact

SEQ ID NO: 12918 - RNA, 20 nt, synthetic construct
  source 1..20: mol_type = other RNA
gcccagttgttggtaggcag

SEQ ID NO: 12919 - RNA, 20 nt, synthetic construct
  source 1..20: mol_type = other RNA
ccaacaactgggcttatcac

SEQ ID NO: 12920 - RNA, 20 nt, synthetic construct
  source 1..20: mol_type = other RNA
caacaactgggcttatcact

SEQ ID NO: 12921 - RNA, 20 nt, synthetic construct
  source 1..20: mol_type = other RNA
ccagtgataagcccagttgt

SEQ ID NO: 12922 - RNA, 20 nt, synthetic construct
  source 1..20: mol_type = other RNA
ctagttcttttgttgttgct

SEQ ID NO: 12923 - RNA, 20 nt, synthetic construct
  source 1..20: mol_type = other RNA
actagttcttttgttgttgc

SEQ ID NO: 12924 - RNA, 20 nt, synthetic construct
  source 1..20: mol_type = other RNA
aaagcgcaagaaattctaag

SEQ ID NO: 12925 - RNA, 20 nt, synthetic construct
  source 1..20: mol_type = other RNA
tcttgcgctttgattttttt

SEQ ID NO: 12926 - RNA, 20 nt, synthetic construct
  source 1..20: mol_type = other RNA
cttgcgctttgattttttta

SEQ ID NO: 12927 - RNA, 20 nt, synthetic construct
  source 1..20: mol_type = other RNA
ttgtgccctgtttcacttat

SEQ ID NO: 12928 - RNA, 20 nt, synthetic construct
  source 1..20: mol_type = other RNA
tgtgccctgtttcacttata

SEQ ID NO: 12929 - RNA, 20 nt, synthetic construct
  source 1..20: mol_type = other RNA
tagaccctataagtgaaaca

SEQ ID NO: 12930 - RNA, 20 nt, synthetic construct
  source 1..20: mol_type = other RNA
ctagaccctataagtgaaac

SEQ ID NO: 12931 - RNA, 20 nt, synthetic construct
  source 1..20: mol_type = other RNA
aatgcttgtgttgagtaaaa

SEQ ID NO: 12932 - RNA, 20 nt, synthetic construct
  source 1..20: mol_type = other RNA
atttagcagctttgaatatt

SEQ ID NO: 12933 - RNA, 20 nt, synthetic construct
  source 1..20: mol_type = other RNA
catttagcagctttgaatat

SEQ ID NO: 12934 - RNA, 20 nt, synthetic construct
  source 1..20: mol_type = other RNA
acagttacacggagtcttta

SEQ ID NO: 12935 - RNA, 20 nt, synthetic construct
  source 1..20: mol_type = other RNA
cgtgtaactgtgtgaacact

SEQ ID NO: 12936 - RNA, 20 nt, synthetic construct
  source 1..20: mol_type = other RNA
gtgtaactgtgtgaacactt

SEQ ID NO: 12937 - RNA, 20 nt, synthetic construct
  source 1..20: mol_type = other RNA
caagtgttcacacagttaca

SEQ ID NO: 12938 - RNA, 20 nt, synthetic construct
  source 1..20: mol_type = other RNA
gatttttctcctctgtcccg

SEQ ID NO: 12939 - RNA, 20 nt, synthetic construct
  source 1..20: mol_type = other RNA
agacgacgacctcgggacag

SEQ ID NO: 12940 - RNA, 20 nt, synthetic construct
  source 1..20: mol_type = other RNA
agaaagcagacgacgacctc

SEQ ID NO: 12941 - RNA, 20 nt, synthetic construct
  source 1..20: mol_type = other RNA
aagaaagcagacgacgacct

SEQ ID NO: 12942 - RNA, 20 nt, synthetic construct
  source 1..20: mol_type = other RNA
tcgtcgtctgctttcttttt

SEQ ID NO: 12943 - RNA, 20 nt, synthetic construct
  source 1..20: mol_type = other RNA
cgtcgtctgctttctttttt

SEQ ID NO: 12944 - RNA, 20 nt, synthetic construct
  source 1..20: mol_type = other RNA
gattgagaagtgcatatgac

SEQ ID NO: 12945 - RNA, 20 nt, synthetic construct
  source 1..20: mol_type = other RNA
gagagcttgtgtgtttgggg

SEQ ID NO: 12946 - RNA, 20 nt, synthetic construct
  source 1..20: mol_type = other RNA
gctgagagcttgtgtgtttg

SEQ ID NO: 12947 - RNA, 20 nt, synthetic construct
  source 1..20: mol_type = other RNA
ggctgagagcttgtgtgttt

SEQ ID NO: 12948 - RNA, 20 nt, synthetic construct
  source 1..20: mol_type = other RNA
tggctgagagcttgtgtgtt

SEQ ID NO: 12949 - RNA, 20 nt, synthetic construct
  source 1..20: mol_type = other RNA
ggctgtggagaagctgcctg

SEQ ID NO: 12950 - RNA, 20 nt, synthetic construct
  source 1..20: mol_type = other RNA
ccacagccccagcttcgcac

SEQ ID NO: 12951 - RNA, 20 nt, synthetic construct
  source 1..20: mol_type = other RNA
cctgtgcgaagctggggctg

SEQ ID NO: 12952 - RNA, 20 nt, synthetic construct
  source 1..20: mol_type = other RNA
cccagcttcgcacaggctcc

SEQ ID NO: 12953 - RNA, 20 nt, synthetic construct
  source 1..20: mol_type = other RNA
agcttcgcacaggctcctgg

SEQ ID NO: 12954 - RNA, 20 nt, synthetic construct
  source 1..20: mol_type = other RNA
caggagcctgtgcgaagctg

SEQ ID NO: 12955 - RNA, 20 nt, synthetic construct
  source 1..20: mol_type = other RNA
ccaggagcctgtgcgaagct

SEQ ID NO: 12956 - RNA, 20 nt, synthetic construct
  source 1..20: mol_type = other RNA
tccaggagcctgtgcgaagc

SEQ ID NO: 12957 - RNA, 20 nt, synthetic construct
  source 1..20: mol_type = other RNA
caggctcctggagggctgcc

SEQ ID NO: 12958 - RNA, 20 nt, synthetic construct
  source 1..20: mol_type = other RNA
aggctcctggagggctgcct

SEQ ID NO: 12959 - RNA, 20 nt, synthetic construct
  source 1..20: mol_type = other RNA
ggctcctggagggctgcctg

SEQ ID NO: 12960 - RNA, 20 nt, synthetic construct
  source 1..20: mol_type = other RNA
gctcctggagggctgcctgg

SEQ ID NO: 12961 - RNA, 20 nt, synthetic construct
  source 1..20: mol_type = other RNA
cctggagggctgcctggggg

SEQ ID NO: 12962 - RNA, 20 nt, synthetic construct
  source 1..20: mol_type = other RNA
cctcccccaggcagccctcc

SEQ ID NO: 12963 - RNA, 20 nt, synthetic construct
  source 1..20: mol_type = other RNA
ctgcctgggggaggcagaca

SEQ ID NO: 12964 - RNA, 20 nt, synthetic construct
  source 1..20: mol_type = other RNA
tgcctgggggaggcagacat

SEQ ID NO: 12965 - RNA, 20 nt, synthetic construct
  source 1..20: mol_type = other RNA
ctcccatgtctgcctccccc

SEQ ID NO: 12966 - RNA, 20 nt, synthetic construct
  source 1..20: mol_type = other RNA
aggcagacatgggagtgcca

SEQ ID NO: 12967 - RNA, 20 nt, synthetic construct
  source 1..20: mol_type = other RNA
cagacatgggagtgccaagg

SEQ ID NO: 12968 - RNA, 20 nt, synthetic construct
  source 1..20: mol_type = other RNA
ggagtgccaaggtggccaga

SEQ ID NO: 12969 - RNA, 20 nt, synthetic construct
  source 1..20: mol_type = other RNA
caaggtggccagatggttcc

SEQ ID NO: 12970 - RNA, 20 nt, synthetic construct
  source 1..20: mol_type = other RNA
ctggaaccatctggccacct

SEQ ID NO: 12971 - RNA, 20 nt, synthetic construct
  source 1..20: mol_type = other RNA
attgtagtcctggaaccatc

SEQ ID NO: 12972 - RNA, 20 nt, synthetic construct
  source 1..20: mol_type = other RNA
aaataaagacattgtagtcc

SEQ ID NO: 12973 - RNA, 20 nt, synthetic construct
  source 1..20: mol_type = other RNA
ctgctgccctcacccctgcc

SEQ ID NO: 12974 - RNA, 20 nt, synthetic construct
  source 1..20: mol_type = other RNA
ggcaggggtgagggcagcag

SEQ ID NO: 12975 - RNA, 20 nt, synthetic construct
  source 1..20: mol_type = other RNA
ccctcacccctgcccggctc

SEQ ID NO: 12976 - RNA, 20 nt, synthetic construct
  source 1..20: mol_type = other RNA
ccagagccgggcaggggtga

SEQ ID NO: 12977 - RNA, 20 nt, synthetic construct
  source 1..20: mol_type = other RNA
tccagagccgggcaggggtg

SEQ ID NO: 12978 - RNA, 20 nt, synthetic construct
  source 1..20: mol_type = other RNA
ggtactccagagccgggcag

SEQ ID NO: 12979 - RNA, 20 nt, synthetic construct
  source 1..20: mol_type = other RNA
cggtactccagagccgggca

SEQ ID NO: 12980 - RNA, 20 nt, synthetic construct
  source 1..20: mol_type = other RNA
acggtactccagagccgggc

SEQ ID NO: 12981 - RNA, 20 nt, synthetic construct
  source 1..20: mol_type = other RNA
gcagacggtactccagagcc

SEQ ID NO: 12982 - RNA, 20 nt, synthetic construct
  source 1..20: mol_type = other RNA
ggcagacggtactccagagc

SEQ ID NO: 12983 - RNA, 20 nt, synthetic construct
  source 1..20: mol_type = other RNA
taccgtctgccccagacaag

SEQ ID NO: 12984 - RNA, 20 nt, synthetic construct
  source 1..20: mol_type = other RNA
accgtctgccccagacaagt

SEQ ID NO: 12985 - RNA, 20 nt, synthetic construct
  source 1..20: mol_type = other RNA
tcccacttgtctggggcaga

SEQ ID NO: 12986 - RNA, 20 nt, synthetic construct
  source 1..20: mol_type = other RNA
ccagacaagtgggagtgaaa

SEQ ID NO: 12987 - RNA, 20 nt, synthetic construct
  source 1..20: mol_type = other RNA
cagacaagtgggagtgaaat

SEQ ID NO: 12988 - RNA, 20 nt, synthetic construct
  source 1..20: mol_type = other RNA
agacaagtgggagtgaaatg

SEQ ID NO: 12989 - RNA, 20 nt, synthetic construct
  source 1..20: mol_type = other RNA
atttcactcccacttgtctg

SEQ ID NO: 12990 - RNA, 20 nt, synthetic construct
  source 1..20: mol_type = other RNA
catttcactcccacttgtct

SEQ ID NO: 12991 - RNA, 20 nt, synthetic construct
  source 1..20: mol_type = other RNA
ccatttcactcccacttgtc

SEQ ID NO: 12992 - RNA, 20 nt, synthetic construct
  source 1..20: mol_type = other RNA
aagtgggagtgaaatggggg

SEQ ID NO: 12993 - RNA, 20 nt, synthetic construct
  source 1..20: mol_type = other RNA
agtgggagtgaaatgggggt

SEQ ID NO: 12994 - RNA, 20 nt, synthetic construct
  source 1..20: mol_type = other RNA
gtgggagtgaaatgggggtg

SEQ ID NO: 12995 - RNA, 20 nt, synthetic construct
  source 1..20: mol_type = other RNA
tgggagtgaaatgggggtgg

SEQ ID NO: 12996 - RNA, 20 nt, synthetic construct
  source 1..20: mol_type = other RNA
gggagtgaaatgggggtggg

SEQ ID NO: 12997 - RNA, 20 nt, synthetic construct
  source 1..20: mol_type = other RNA
ggaagcactgattcccagtt

SEQ ID NO: 12998 - RNA, 20 nt, synthetic construct
  source 1..20: mol_type = other RNA
gaagcactgattcccagtta

SEQ ID NO: 12999 - RNA, 20 nt, synthetic construct
  source 1..20: mol_type = other RNA
aagcactgattcccagttag

SEQ ID NO: 13000 - RNA, 20 nt, synthetic construct
  source 1..20: mol_type = other RNA
agcactgattcccagttagg

SEQ ID NO: 13001 - RNA, 20 nt, synthetic construct
  source 1..20: mol_type = other RNA
cagttaggcaccccctaact

SEQ ID NO: 13002 - RNA, 20 nt, synthetic construct
  source 1..20: mol_type = other RNA
tcagttaggcaccccctaac

SEQ ID NO: 13003 - RNA, 20 nt, synthetic construct
  source 1..20: mol_type = other RNA
ggggtgcctaactgagcagt

SEQ ID NO: 13004 - RNA, 20 nt, synthetic construct
  source 1..20: mol_type = other RNA
gggtgcctaactgagcagta

SEQ ID NO: 13005 - RNA, 20 nt, synthetic construct
  source 1..20: mol_type = other RNA
aactgagcagtagggataga

SEQ ID NO: 13006 - RNA, 20 nt, synthetic construct
  source 1..20: mol_type = other RNA
tctatccctactgctcagtt

SEQ ID NO: 13007 - RNA, 20 nt, synthetic construct
  source 1..20: mol_type = other RNA
agggatagaaggtgtgaacc

SEQ ID NO: 13008 - RNA, 20 nt, synthetic construct
  source 1..20: mol_type = other RNA
gggatagaaggtgtgaacct

SEQ ID NO: 13009 - RNA, 20 nt, synthetic construct
  source 1..20: mol_type = other RNA
taatttataaaagcactccc

SEQ ID NO: 13010 - RNA, 20 nt, synthetic construct
  source 1..20: mol_type = other RNA
aattaaaaataaaatctaca

SEQ ID NO: 13011 - RNA, 20 nt, synthetic construct
  source 1..20: mol_type = other RNA
atttatctctgtgacctgcc

SEQ ID NO: 13012 - RNA, 20 nt, synthetic construct
  source 1..20: mol_type = other RNA
tttatctctgtgacctgcca

SEQ ID NO: 13013 - RNA, 20 nt, synthetic construct
  source 1..20: mol_type = other RNA
ctctgtgacctgccagggag

SEQ ID NO: 13014 - RNA, 20 nt, synthetic construct
  source 1..20: mol_type = other RNA
tctgtgacctgccagggaga

SEQ ID NO: 13015 - RNA, 20 nt, synthetic construct
  source 1..20: mol_type = other RNA
ctgtgacctgccagggagag

SEQ ID NO: 13016 - RNA, 20 nt, synthetic construct
  source 1..20: mol_type = other RNA
ctctctcccctctccctggc

SEQ ID NO: 13017 - RNA, 20 nt, synthetic construct
  source 1..20: mol_type = other RNA
ctctctctctcccctctccc

SEQ ID NO: 13018 - RNA, 20 nt, synthetic construct
  source 1..20: mol_type = other RNA
catgacaaaataaaataaaa

SEQ ID NO: 13019 - RNA, 20 nt, synthetic construct
  source 1..20: mol_type = other RNA
ctcaatttaaattcaaagtg

SEQ ID NO: 13020 - RNA, 20 nt, synthetic construct
  source 1..20: mol_type = other RNA
tctcaatttaaattcaaagt

SEQ ID NO: 13021 - RNA, 20 nt, synthetic construct
  source 1..20: mol_type = other RNA
ttctcaatttaaattcaaag

SEQ ID NO: 13022 - RNA, 20 nt, synthetic construct
  source 1..20: mol_type = other RNA
tgaatttaaattgagaataa

SEQ ID NO: 13023 - RNA, 20 nt, synthetic construct
  source 1..20: mol_type = other RNA
taaattgagaataaaggaaa

SEQ ID NO: 13024 - RNA, 20 nt, synthetic construct
  source 1..20: mol_type = other RNA
aaaggaaatggactcattgt

SEQ ID NO: 13025 - RNA, 20 nt, synthetic construct
  source 1..20: mol_type = other RNA
atttttgcaaaataaagtga

SEQ ID NO: 13026 - RNA, 20 nt, synthetic construct
  source 1..20: mol_type = other RNA
ctcagcaatatgcgatacag

SEQ ID NO: 13027 - RNA, 20 nt, synthetic construct
  source 1..20: mol_type = other RNA
tcagcaatatgcgatacagc

SEQ ID NO: 13028 - RNA, 20 nt, synthetic construct
  source 1..20: mol_type = other RNA
cagcaatatgcgatacagcg

SEQ ID NO: 13029 - RNA, 20 nt, synthetic construct
  source 1..20: mol_type = other RNA
tatgcgatacagcggggtag

SEQ ID NO: 13030 - RNA, 20 nt, synthetic construct
  source 1..20: mol_type = other RNA
atgcgatacagcggggtaga

SEQ ID NO: 13031 - RNA, 20 nt, synthetic construct
  source 1..20: mol_type = other RNA
tgcgatacagcggggtagag

SEQ ID NO: 13032 - RNA, 20 nt, synthetic construct
  source 1..20: mol_type = other RNA
tagaggggagatgtaaacag

SEQ ID NO: 13033 - RNA, 20 nt, synthetic construct
  source 1..20: mol_type = other RNA
agaggggagatgtaaacaga

SEQ ID NO: 13034 - RNA, 20 nt, synthetic construct
  source 1..20: mol_type = other RNA
gaggggagatgtaaacagag

SEQ ID NO: 13035 - RNA, 20 nt, synthetic construct
  source 1..20: mol_type = other RNA
gggagatgtaaacagagggg

SEQ ID NO: 13036 - RNA, 20 nt, synthetic construct
  source 1..20: mol_type = other RNA
ggagatgtaaacagagggga

SEQ ID NO: 13037 - RNA, 20 nt, synthetic construct
  source 1..20: mol_type = other RNA
gagatgtaaacagaggggag

SEQ ID NO: 13038 - RNA, 20 nt, synthetic construct
  source 1..20: mol_type = other RNA
ctgaccccccaagagaacac

SEQ ID NO: 13039 - RNA, 20 nt, synthetic construct
  source 1..20: mol_type = other RNA
tgaccccccaagagaacaca

SEQ ID NO: 13040 - RNA, 20 nt, synthetic construct
  source 1..20: mol_type = other RNA
tgtgttctcttggggggtca

SEQ ID NO: 13041 - RNA, 20 nt, synthetic construct
  source 1..20: mol_type = other RNA
ctgtgttctcttggggggtc

SEQ ID NO: 13042 - RNA, 20 nt, synthetic construct
  source 1..20: mol_type = other RNA
gctccctgtgttctcttggg

SEQ ID NO: 13043 - RNA, 20 nt, synthetic construct
  source 1..20: mol_type = other RNA
ggctccctgtgttctcttgg

SEQ ID NO: 13044 - RNA, 20 nt, synthetic construct
  source 1..20: mol_type = other RNA
tggctccctgtgttctcttg

SEQ ID NO: 13045 - RNA, 20 nt, synthetic construct
  source 1..20: mol_type = other RNA
ttggctccctgtgttctctt

SEQ ID NO: 13046 - RNA, 20 nt, synthetic construct
  source 1..20: mol_type = other RNA
attggctccctgtgttctct

SEQ ID NO: 13047 - RNA, 20 nt, synthetic construct
  source 1..20: mol_type = other RNA
gagccaatgggaatcttatt

SEQ ID NO: 13048 - RNA, 20 nt, synthetic construct
  source 1..20: mol_type = other RNA
ctgccaaataagattcccat

SEQ ID NO: 13049 - RNA, 20 nt, synthetic construct
  source 1..20: mol_type = other RNA
tttggcagctaaatacaaac

SEQ ID NO: 13050 - RNA, 20 nt, synthetic construct
  source 1..20: mol_type = other RNA
ttggcagctaaatacaaact

SEQ ID NO: 13051 - RNA, 20 nt, synthetic construct
  source 1..20: mol_type = other RNA
tggcagctaaatacaaactg

SEQ ID NO: 13052 - RNA, 20 nt, synthetic construct
  source 1..20: mol_type = other RNA
gctaaatacaaactggggat

SEQ ID NO: 13053 - RNA, 20 nt, synthetic construct
  source 1..20: mol_type = other RNA
aaatacaaactggggattgg

SEQ ID NO: 13054 - RNA, 20 nt, synthetic construct
  source 1..20: mol_type = other RNA
actggggattggaggaagaa

SEQ ID NO: 13055 - RNA, 20 nt, synthetic construct
  source 1..20: mol_type = other RNA
ggggattggaggaagaaagg

SEQ ID NO: 13056 - RNA, 20 nt, synthetic construct
  source 1..20: mol_type = other RNA
gggattggaggaagaaagga

SEQ ID NO: 13057 - RNA, 20 nt, synthetic construct
  source 1..20: mol_type = other RNA
ggattggaggaagaaaggag

SEQ ID NO: 13058 - RNA, 20 nt, synthetic construct
  source 1..20: mol_type = other RNA
aggaagaaaggaggggtcac

SEQ ID NO: 13059 - RNA, 20 nt, synthetic construct
  source 1..20: mol_type = other RNA
ggaagaaaggaggggtcaca

SEQ ID NO: 13060 - RNA, 20 nt, synthetic construct
  source 1..20: mol_type = other RNA
gaagaaaggaggggtcacag

SEQ ID NO: 13061 - RNA, 20 nt, synthetic construct
  source 1..20: mol_type = other RNA
aggaggggtcacaggggccc

SEQ ID NO: 13062 - RNA, 20 nt, synthetic construct
  source 1..20: mol_type = other RNA
ggaggggtcacaggggccct

SEQ ID NO: 13063 - RNA, 20 nt, synthetic construct
  source 1..20: mol_type = other RNA
gtcttgggtgggggagccca

SEQ ID NO: 13064 - RNA, 20 nt, synthetic construct
  source 1..20: mol_type = other RNA
gctcccccacccaagacccc

SEQ ID NO: 13065 - RNA, 20 nt, synthetic construct
  source 1..20: mol_type = other RNA
cccccacccaagacccctgg

SEQ ID NO: 13066 - RNA, 20 nt, synthetic construct
  source 1..20: mol_type = other RNA
cacccaagacccctggagga

SEQ ID NO: 13067 - RNA, 20 nt, synthetic construct
  source 1..20: mol_type = other RNA
cctccaggggtcttgggtgg

SEQ ID NO: 13068 - RNA, 20 nt, synthetic construct
  source 1..20: mol_type = other RNA
cccaagacccctggaggaag

SEQ ID NO: 13069 - RNA, 20 nt, synthetic construct
  source 1..20: mol_type = other RNA
ttcctccaggggtcttgggt

SEQ ID NO: 13070 - RNA, 20 nt, synthetic construct
  source 1..20: mol_type = other RNA
cttcctccaggggtcttggg

SEQ ID NO: 13071 - RNA, 20 nt, synthetic construct
  source 1..20: mol_type = other RNA
ccccttcctccaggggtctt

SEQ ID NO: 13072 - RNA, 20 nt, synthetic construct
  source 1..20: mol_type = other RNA
accccttcctccaggggtct

SEQ ID NO: 13073 - RNA, 20 nt, synthetic construct
  source 1..20: mol_type = other RNA
gaattgaccccttcctccag

SEQ ID NO: 13074 - RNA, 20 nt, synthetic construct
  source 1..20: mol_type = other RNA
ggaattgaccccttcctcca

SEQ ID NO: 13075 - RNA, 20 nt, synthetic construct
  source 1..20: mol_type = other RNA
tggaattgaccccttcctcc

SEQ ID NO: 13076 - RNA, 20 nt, synthetic construct
  source 1..20: mol_type = other RNA
attagcttttgtttacaccg

SEQ ID NO: 13077 - RNA, 20 nt, synthetic construct
  source 1..20: mol_type = other RNA
aaaagctaataaataaatag

SEQ ID NO: 13078 - RNA, 20 nt, synthetic construct
  source 1..20: mol_type = other RNA
aaataaatagaggcttcctc

SEQ ID NO: 13079 - RNA, 20 nt, synthetic construct
  source 1..20: mol_type = other RNA
aataaatagaggcttcctct

SEQ ID NO: 13080 - RNA, 20 nt, synthetic construct
  source 1..20: mol_type = other RNA
atagaggcttcctctgggtc

SEQ ID NO: 13081 - RNA, 20 nt, synthetic construct
  source 1..20: mol_type = other RNA
tagaggcttcctctgggtca

SEQ ID NO: 13082 - RNA, 20 nt, synthetic construct
  source 1..20: mol_type = other RNA
aggcttcctctgggtcaggg

SEQ ID NO: 13083 - RNA, 20 nt, synthetic construct
  source 1..20: mol_type = other RNA
ggcttcctctgggtcagggc

SEQ ID NO: 13084 - RNA, 20 nt, synthetic construct
  source 1..20: mol_type = other RNA
ctgatcccgccctgacccag

SEQ ID NO: 13085 - RNA, 20 nt, synthetic construct
  source 1..20: mol_type = other RNA
taagcagcatcccccctccc

SEQ ID NO: 13086 - RNA, 20 nt, synthetic construct
  source 1..20: mol_type = other RNA
aagcagcatcccccctccct

SEQ ID NO: 13087 - RNA, 20 nt, synthetic construct
  source 1..20: mol_type = other RNA
ctccctgggccaagctgctc

SEQ ID NO: 13088 - RNA, 20 nt, synthetic construct
  source 1..20: mol_type = other RNA
tccctgggccaagctgctct

SEQ ID NO: 13089 - RNA, 20 nt, synthetic construct
  source 1..20: mol_type = other RNA
ccctgggccaagctgctctg

SEQ ID NO: 13090 - RNA, 20 nt, synthetic construct
  source 1..20: mol_type = other RNA
agagcagcttggcccaggga

SEQ ID NO: 13091 - RNA, 20 nt, synthetic construct
  source 1..20: mol_type = other RNA
cagagcagcttggcccaggg

SEQ ID NO: 13092 - RNA, 20 nt, synthetic construct
  source 1..20: mol_type = other RNA
ccccagagcagcttggccca

SEQ ID NO: 13093 - RNA, 20 nt, synthetic construct
  source 1..20: mol_type = other RNA
tccccagagcagcttggccc

SEQ ID NO: 13094 - RNA, 20 nt, synthetic construct
  source 1..20: mol_type = other RNA
caagctgctctggggagtaa

SEQ ID NO: 13095 - RNA, 20 nt, synthetic construct
  source 1..20: mol_type = other RNA
aagctgctctggggagtaaa

SEQ ID NO: 13096 - RNA, 20 nt, synthetic construct
  source 1..20: mol_type = other RNA
ctttactccccagagcagct

SEQ ID NO: 13097 - RNA, 20 nt, synthetic construct
  source 1..20: mol_type = other RNA
tctggggagtaaagggtgga

SEQ ID NO: 13098 - RNA, 20 nt, synthetic construct
  source 1..20: mol_type = other RNA
agtaaagggtggaaggcact

SEQ ID NO: 13099 - RNA, 20 nt, synthetic construct
  source 1..20: mol_type = other RNA
gtaaagggtggaaggcacta

SEQ ID NO: 13100 - RNA, 20 nt, synthetic construct
  source 1..20: mol_type = other RNA
gtggaaggcactagggagag

SEQ ID NO: 13101 - RNA, 20 nt, synthetic construct
  source 1..20: mol_type = other RNA
tggaaggcactagggagaga

SEQ ID NO: 13102 - RNA, 20 nt, synthetic construct
  source 1..20: mol_type = other RNA
ctagggagagagggatcccc

SEQ ID NO: 13103 - RNA, 20 nt, synthetic construct
  source 1..20: mol_type = other RNA
ccctggcccctctgtagtgt

SEQ ID NO: 13104 - RNA, 20 nt, synthetic construct
  source 1..20: mol_type = other RNA
tggcccctctgtagtgtagg

SEQ ID NO: 13105 - RNA, 20 nt, synthetic construct
  source 1..20: mol_type = other RNA
ggcccctctgtagtgtagga

SEQ ID NO: 13106 - RNA, 20 nt, synthetic construct
  source 1..20: mol_type = other RNA
cctacactacagaggggcca

SEQ ID NO: 13107 - RNA, 20 nt, synthetic construct
  source 1..20: mol_type = other RNA
tcctacactacagaggggcc

SEQ ID NO: 13108 - RNA, 20 nt, synthetic construct
  source 1..20: mol_type = other RNA
gaccctcctacactacagag

SEQ ID NO: 13109 - RNA, 20 nt, synthetic construct
  source 1..20: mol_type = other RNA
ggaccctcctacactacaga

SEQ ID NO: 13110 - RNA, 20 nt, synthetic construct
  source 1..20: mol_type = other RNA
gggaccctcctacactacag

SEQ ID NO: 13111 - RNA, 20 nt, synthetic construct
  source 1..20: mol_type = other RNA
taggagggtccctgccccaa

SEQ ID NO: 13112 - RNA, 20 nt, synthetic construct
  source 1..20: mol_type = other RNA
ccctgccccaatggctgaga

SEQ ID NO: 13113 - RNA, 20 nt, synthetic construct
  source 1..20: mol_type = other RNA
tgccccaatggctgagatgg

SEQ ID NO: 13114 - RNA, 20 nt, synthetic construct
  source 1..20: mol_type = other RNA
gccccaatggctgagatgga

SEQ ID NO: 13115 - RNA, 20 nt, synthetic construct
  source 1..20: mol_type = other RNA
ccatctcagccattggggca

SEQ ID NO: 13116 - RNA, 20 nt, synthetic construct
  source 1..20: mol_type = other RNA
tccatctcagccattggggc

SEQ ID NO: 13117 - RNA, 20 nt, synthetic construct
  source 1..20: mol_type = other RNA
caatggctgagatggagggc

SEQ ID NO: 13118 - RNA, 20 nt, synthetic construct
  source 1..20: mol_type = other RNA
gccctccatctcagccattg

SEQ ID NO: 13119 - RNA, 20 nt, synthetic construct
  source 1..20: mol_type = other RNA
tgccctccatctcagccatt

SEQ ID NO: 13120 - RNA, 20 nt, synthetic construct
  source 1..20: mol_type = other RNA
ctgccctccatctcagccat

SEQ ID NO: 13121 - RNA, 20 nt, synthetic construct
  source 1..20: mol_type = other RNA
tggagggcaggaggagccca

SEQ ID NO: 13122 - RNA, 20 nt, synthetic construct
  source 1..20: mol_type = other RNA
aggagcccaaggcacatgac

SEQ ID NO: 13123 - RNA, 20 nt, synthetic construct
  source 1..20: mol_type = other RNA
ggagcccaaggcacatgaca

SEQ ID NO: 13124 - RNA, 20 nt, synthetic construct
  source 1..20: mol_type = other RNA
cccaaggcacatgacagggc

SEQ ID NO: 13125 - RNA, 20 nt, synthetic construct
  source 1..20: mol_type = other RNA
ccaaggcacatgacagggct

SEQ ID NO: 13126 - RNA, 20 nt, synthetic construct
  source 1..20: mol_type = other RNA
caaggcacatgacagggctg

SEQ ID NO: 13127 - RNA, 20 nt, synthetic construct
  source 1..20: mol_type = other RNA
aaggcacatgacagggctgg

SEQ ID NO: 13128 - RNA, 20 nt, synthetic construct
  source 1..20: mol_type = other RNA
ccagccctgtcatgtgcctt

SEQ ID NO: 13129 - RNA, 20 nt, synthetic construct
  source 1..20: mol_type = other RNA
gcacatgacagggctggggg

SEQ ID NO: 13130 - RNA, 20 nt, synthetic construct
  source 1..20: mol_type = other RNA
cacatgacagggctggggga

SEQ ID NO: 13131 - RNA, 20 nt, synthetic construct
  source 1..20: mol_type = other RNA
gctgggggagggacttataa

SEQ ID NO: 13132 - RNA, 20 nt, synthetic construct
  source 1..20: mol_type = other RNA
gggggagggacttataacgg

SEQ ID NO: 13133 - RNA, 20 nt, synthetic construct
  source 1..20: mol_type = other RNA
ggggagggacttataacgga

SEQ ID NO: 13134 - RNA, 20 nt, synthetic construct
  source 1..20: mol_type = other RNA
ggacttataacggagggcac

SEQ ID NO: 13135 - RNA, 20 nt, synthetic construct
  source 1..20: mol_type = other RNA
gacttataacggagggcaca

SEQ ID NO: 13136 - RNA, 20 nt, synthetic construct
  source 1..20: mol_type = other RNA
aactctgcacccgagccaag

SEQ ID NO: 13137 - RNA, 20 nt, synthetic construct
  source 1..20: mol_type = other RNA
ccgagccaagaggtgcagaa

SEQ ID NO: 13138 - RNA, 20 nt, synthetic construct
  source 1..20: mol_type = other RNA
cattctgcacctcttggctc

SEQ ID NO: 13139 - RNA, 20 nt, synthetic construct
  source 1..20: mol_type = other RNA
ccattctgcacctcttggct

SEQ ID NO: 13140 - RNA, 20 nt, synthetic construct
  source 1..20: mol_type = other RNA
caggtccattctgcacctct

SEQ ID NO: 13141 - RNA, 20 nt, synthetic construct
  source 1..20: mol_type = other RNA
tgaaagggacagatagatgc

SEQ ID NO: 13142 - RNA, 20 nt, synthetic construct
  source 1..20: mol_type = other RNA
ggcaggaacagagggtgaaa

SEQ ID NO: 13143 - RNA, 20 nt, synthetic construct
  source 1..20: mol_type = other RNA
gggcaggaacagagggtgaa

SEQ ID NO: 13144 - RNA, 20 nt, synthetic construct
  source 1..20: mol_type = other RNA
tgttcctgccccagaaatgc

SEQ ID NO: 13145 - RNA, 20 nt, synthetic construct
  source 1..20: mol_type = other RNA
gttcctgccccagaaatgca

SEQ ID NO: 13146 - RNA, 20 nt, synthetic construct
  source 1..20: mol_type = other RNA
gggccctgcatttctggggc

SEQ ID NO: 13147 - RNA, 20 nt, synthetic construct
  source 1..20: mol_type = other RNA
ggctgggccctgcatttctg

SEQ ID NO: 13148 - RNA, 20 nt, synthetic construct
  source 1..20: mol_type = other RNA
aggctgggccctgcatttct

SEQ ID NO: 13149 - RNA, 20 nt, synthetic construct
  source 1..20: mol_type = other RNA
caggctgggccctgcatttc

SEQ ID NO: 13150 - RNA, 20 nt, synthetic construct
  source 1..20: mol_type = other RNA
agcctgcccccaccttgacc

SEQ ID NO: 13151 - RNA, 20 nt, synthetic construct
  source 1..20: mol_type = other RNA
ggtcaaggtgggggcaggct

SEQ ID NO: 13152 - RNA, 20 nt, synthetic construct
  source 1..20: mol_type = other RNA
aggtcaaggtgggggcaggc

SEQ ID NO: 13153 - RNA, 20 nt, synthetic construct
  source 1..20: mol_type = other RNA
tgccaggtcaaggtgggggc

SEQ ID NO: 13154 - RNA, 20 nt, synthetic construct
  source 1..20: mol_type = other RNA
cttgtgccaggtcaaggtgg

SEQ ID NO: 13155 - RNA, 20 nt, synthetic construct
  source 1..20: mol_type = other RNA
ccttgtgccaggtcaaggtg

SEQ ID NO: 13156 - RNA, 20 nt, synthetic construct
  source 1..20: mol_type = other RNA
cttgacctggcacaaggacg

SEQ ID NO: 13157 - RNA, 20 nt, synthetic construct
  source 1..20: mol_type = other RNA
gtccttgtgccaggtcaagg

SEQ ID NO: 13158 - RNA, 20 nt, synthetic construct
  source 1..20: mol_type = other RNA
cccgtccttgtgccaggtca

SEQ ID NO: 13159 - RNA, 20 nt, synthetic construct
  source 1..20: mol_type = other RNA
ggcacaaggacggggcacag

SEQ ID NO: 13160 - RNA, 20 nt, synthetic construct
  source 1..20: mol_type = other RNA
ctgtgccccgtccttgtgcc

SEQ ID NO: 13161 - RNA, 20 nt, synthetic construct
  source 1..20: mol_type = other RNA
gaggctagcacacaccctgc

SEQ ID NO: 13162 - RNA, 20 nt, synthetic construct
  source 1..20: mol_type = other RNA
tgctgtgtgatgcacctgca

SEQ ID NO: 13163 - RNA, 20 nt, synthetic construct
  source 1..20: mol_type = other RNA
atgctgtgtgatgcacctgc

SEQ ID NO: 13164 - RNA, 20 nt, synthetic construct
  source 1..20: mol_type = other RNA
tcacacagcattaggcacca

SEQ ID NO: 13165 - RNA, 20 nt, synthetic construct
  source 1..20: mol_type = other RNA
cacacagcattaggcaccaa

SEQ ID NO: 13166 - RNA, 20 nt, synthetic construct
  source 1..20: mol_type = other RNA
cagcattaggcaccaagggt

SEQ ID NO: 13167 - RNA, 20 nt, synthetic construct
  source 1..20: mol_type = other RNA
caccaagggtaggagcaaga

SEQ ID NO: 13168 - RNA, 20 nt, synthetic construct
  source 1..20: mol_type = other RNA
caagggtaggagcaagaagg

SEQ ID NO: 13169 - RNA, 20 nt, synthetic construct
  source 1..20: mol_type = other RNA
aagggtaggagcaagaaggt

SEQ ID NO: 13170 - RNA, 20 nt, synthetic construct
  source 1..20: mol_type = other RNA
caccttcttgctcctaccct

SEQ ID NO: 13171 - RNA, 20 nt, synthetic construct
  source 1..20: mol_type = other RNA
cttctcctttgtcccctttt

SEQ ID NO: 13172 - RNA, 20 nt, synthetic construct
  source 1..20: mol_type = other RNA
aaaaaggggacaaaggagaa

SEQ ID NO: 13173 - RNA, 20 nt, synthetic construct
  source 1..20: mol_type = other RNA
caaaaaggggacaaaggaga

SEQ ID NO: 13174 - RNA, 20 nt, synthetic construct
  source 1..20: mol_type = other RNA
agagaccaaaaaggggacaa

SEQ ID NO: 13175 - RNA, 20 nt, synthetic construct
  source 1..20: mol_type = other RNA
gaacactagagaccaaaaag

SEQ ID NO: 13176 - RNA, 20 nt, synthetic construct
  source 1..20: mol_type = other RNA
ggaacactagagaccaaaaa

SEQ ID NO: 13177 - RNA, 20 nt, synthetic construct
  source 1..20: mol_type = other RNA
aggaacactagagaccaaaa

SEQ ID NO: 13178 - RNA, 20 nt, synthetic construct
  source 1..20: mol_type = other RNA
ttggctctctgagagcaaac

SEQ ID NO: 13179 - RNA, 20 nt, synthetic construct
  source 1..20: mol_type = other RNA
ctctcagagagccaagcacc

SEQ ID NO: 13180 - RNA, 20 nt, synthetic construct
  source 1..20: mol_type = other RNA
gagagccaagcacctggcag

SEQ ID NO: 13181 - RNA, 20 nt, synthetic construct
  source 1..20: mol_type = other RNA
gccaagcacctggcagagga

SEQ ID NO: 13182 - RNA, 20 nt, synthetic construct
  source 1..20: mol_type = other RNA
ccaagcacctggcagaggaa

SEQ ID NO: 13183 - RNA, 20 nt, synthetic construct
  source 1..20: mol_type = other RNA
caagcacctggcagaggaag

SEQ ID NO: 13184 - RNA, 20 nt, synthetic construct
  source 1..20: mol_type = other RNA
cccttcctctgccaggtgct

SEQ ID NO: 13185 - RNA, 20 nt, synthetic construct
  source 1..20: mol_type = other RNA
cctggcagaggaaggggctg

SEQ ID NO: 13186 - RNA, 20 nt, synthetic construct
  source 1..20: mol_type = other RNA
ccacagccccttcctctgcc

SEQ ID NO: 13187 - RNA, 20 nt, synthetic construct
  source 1..20: mol_type = other RNA
ggaaggggctgtggaatggc

SEQ ID NO: 13188 - RNA, 20 nt, synthetic construct
  source 1..20: mol_type = other RNA
gaaggggctgtggaatggca

SEQ ID NO: 13189 - RNA, 20 nt, synthetic construct
  source 1..20: mol_type = other RNA
gcagggtcttcctcttgccc

SEQ ID NO: 13190 - RNA, 20 nt, synthetic construct
  source 1..20: mol_type = other RNA
cagggtcttcctcttgccct

SEQ ID NO: 13191 - RNA, 20 nt, synthetic construct
  source 1..20: mol_type = other RNA
cctcttgccctgggaagtct

SEQ ID NO: 13192 - RNA, 20 nt, synthetic construct
  source 1..20: mol_type = other RNA
cctagacttcccagggcaag

SEQ ID NO: 13193 - RNA, 20 nt, synthetic construct
  source 1..20: mol_type = other RNA
cctgggaagtctaggaccca

SEQ ID NO: 13194 - RNA, 20 nt, synthetic construct
  source 1..20: mol_type = other RNA
ctgggaagtctaggacccat

SEQ ID NO: 13195 - RNA, 20 nt, synthetic construct
  source 1..20: mol_type = other RNA
tgggaagtctaggacccatg

SEQ ID NO: 13196 - RNA, 20 nt, synthetic construct
  source 1..20: mol_type = other RNA
catgggtcctagacttccca

SEQ ID NO: 13197 - RNA, 20 nt, synthetic construct
  source 1..20: mol_type = other RNA
ccatgggtcctagacttccc

SEQ ID NO: 13198 - RNA, 20 nt, synthetic construct
  source 1..20: mol_type = other RNA
aaatctcagcactgccccat

SEQ ID NO: 13199 - RNA, 20 nt, synthetic construct
  source 1..20: mol_type = other RNA
aaaatctcagcactgcccca

SEQ ID NO: 13200 - RNA, 20 nt, synthetic construct
  source 1..20: mol_type = other RNA
agattttagagtccaaaccc

SEQ ID NO: 13201 - RNA, 20 nt, synthetic construct
  source 1..20: mol_type = other RNA
caaagggatgagcctgggtt

SEQ ID NO: 13202 - RNA, 20 nt, synthetic construct
  source 1..20: mol_type = other RNA
gagggcaaagggatgagcct

SEQ ID NO: 13203 - RNA, 20 nt, synthetic construct
  source 1..20: mol_type = other RNA
agagggcaaagggatgagcc

SEQ ID NO: 13204 - RNA, 20 nt, synthetic construct
  source 1..20: mol_type = other RNA
catccctttgccctctctcc

SEQ ID NO: 13205 - RNA, 20 nt, synthetic construct
  source 1..20: mol_type = other RNA
ccctttgccctctctcctgg

SEQ ID NO: 13206 - RNA, 20 nt, synthetic construct
  source 1..20: mol_type = other RNA
cctttgccctctctcctggt

SEQ ID NO: 13207 - RNA, 20 nt, synthetic construct
  source 1..20: mol_type = other RNA
ccaccaggagagagggcaaa

SEQ ID NO: 13208 - RNA, 20 nt, synthetic construct
  source 1..20: mol_type = other RNA
cccaccaggagagagggcaa

SEQ ID NO: 13209 - RNA, 20 nt, synthetic construct
  source 1..20: mol_type = other RNA
ccctctctcctggtgggagc

SEQ ID NO: 13210 - RNA, 20 nt, synthetic construct
  source 1..20: mol_type = other RNA
cctctctcctggtgggagca

SEQ ID NO: 13211 - RNA, 20 nt, synthetic construct
  source 1..20: mol_type = other RNA
cctgctcccaccaggagaga

SEQ ID NO: 13212 - RNA, 20 nt, synthetic construct
  source 1..20: mol_type = other RNA
ccctgctcccaccaggagag

SEQ ID NO: 13213 - RNA, 20 nt, synthetic construct
  source 1..20: mol_type = other RNA
gtgggagcagggcaggcccc

SEQ ID NO: 13214 - RNA, 20 nt, synthetic construct
  source 1..20: mol_type = other RNA
tgggagcagggcaggccccc

SEQ ID NO: 13215 - RNA, 20 nt, synthetic construct
  source 1..20: mol_type = other RNA
gcagggcaggcccccgggac

SEQ ID NO: 13216 - RNA, 20 nt, synthetic construct
  source 1..20: mol_type = other RNA
gcaggcccccgggactggcg

SEQ ID NO: 13217 - RNA, 20 nt, synthetic construct
  source 1..20: mol_type = other RNA
caggcccccgggactggcga

SEQ ID NO: 13218 - RNA, 20 nt, synthetic construct
  source 1..20: mol_type = other RNA
cccgggactggcgagggagc

SEQ ID NO: 13219 - RNA, 20 nt, synthetic construct
  source 1..20: mol_type = other RNA
ggctccctcgccagtcccgg

SEQ ID NO: 13220 - RNA, 20 nt, synthetic construct
  source 1..20: mol_type = other RNA
cggctccctcgccagtcccg

SEQ ID NO: 13221 - RNA, 20 nt, synthetic construct
  source 1..20: mol_type = other RNA
ccggctccctcgccagtccc

SEQ ID NO: 13222 - RNA, 20 nt, synthetic construct
  source 1..20: mol_type = other RNA
accggctccctcgccagtcc

SEQ ID NO: 13223 - RNA, 20 nt, synthetic construct
  source 1..20: mol_type = other RNA
gcgagggagccggttagatc

SEQ ID NO: 13224 - RNA, 20 nt, synthetic construct
  source 1..20: mol_type = other RNA
gggagccggttagatcagga

SEQ ID NO: 13225 - RNA, 20 nt, synthetic construct
  source 1..20: mol_type = other RNA
ggagccggttagatcaggaa

SEQ ID NO: 13226 - RNA, 20 nt, synthetic construct
  source 1..20: mol_type = other RNA
gagccggttagatcaggaag

SEQ ID NO: 13227 - RNA, 20 nt, synthetic construct
  source 1..20: mol_type = other RNA
catccccttcctgatctaac

SEQ ID NO: 13228 - RNA, 20 nt, synthetic construct
  source 1..20: mol_type = other RNA
caggaaggggatgaacacag

SEQ ID NO: 13229 - RNA, 20 nt, synthetic construct
  source 1..20: mol_type = other RNA
agaggcacccctagaaactt

SEQ ID NO: 13230 - RNA, 20 nt, synthetic construct
  source 1..20: mol_type = other RNA
tagaaactttggcaaaaaca

SEQ ID NO: 13231 - RNA, 20 nt, synthetic construct
  source 1..20: mol_type = other RNA
gtttttgccaaagtttctag

SEQ ID NO: 13232 - RNA, 20 nt, synthetic construct
  source 1..20: mol_type = other RNA
tgtttttgccaaagtttcta

SEQ ID NO: 13233 - RNA, 20 nt, synthetic construct
  source 1..20: mol_type = other RNA
ttgtttttgccaaagtttct

SEQ ID NO: 13234 - RNA, 20 nt, synthetic construct
  source 1..20: mol_type = other RNA
ggcaaaaacaaggagctcat

SEQ ID NO: 13235 - RNA, 20 nt, synthetic construct
  source 1..20: mol_type = other RNA
aaaacaaggagctcattgga

SEQ ID NO: 13236 - RNA, 20 nt, synthetic construct
  source 1..20: mol_type = other RNA
aaacaaggagctcattggaa

SEQ ID NO: 13237 - RNA, 20 nt, synthetic construct
  source 1..20: mol_type = other RNA
aacaaggagctcattggaag

SEQ ID NO: 13238 - RNA, 20 nt, synthetic construct
  source 1..20: mol_type = other RNA
aaggagctcattggaagggg

SEQ ID NO: 13239 - RNA, 20 nt, synthetic construct
  source 1..20: mol_type = other RNA
aggagctcattggaaggggt

SEQ ID NO: 13240 - RNA, 20 nt, synthetic construct
  source 1..20: mol_type = other RNA
ggagctcattggaaggggtg

SEQ ID NO: 13241 - RNA, 20 nt, synthetic construct
  source 1..20: mol_type = other RNA
tcattggaaggggtggggag

SEQ ID NO: 13242 - RNA, 20 nt, synthetic construct
  source 1..20: mol_type = other RNA
cattggaaggggtggggaga

SEQ ID NO: 13243 - RNA, 20 nt, synthetic construct
  source 1..20: mol_type = other RNA
gggtggggagagggcagagc

SEQ ID NO: 13244 - RNA, 20 nt, synthetic construct
  source 1..20: mol_type = other RNA
gcaggtcctcccccagtcac

SEQ ID NO: 13245 - RNA, 20 nt, synthetic construct
  source 1..20: mol_type = other RNA
ggtcctcccccagtcactgg

SEQ ID NO: 13246 - RNA, 20 nt, synthetic construct
  source 1..20: mol_type = other RNA
tcccccagtcactggcggtc

SEQ ID NO: 13247 - RNA, 20 nt, synthetic construct
  source 1..20: mol_type = other RNA
cccccagtcactggcggtct

SEQ ID NO: 13248 - RNA, 20 nt, synthetic construct
  source 1..20: mol_type = other RNA
agaccgccagtgactggggg

SEQ ID NO: 13249 - RNA, 20 nt, synthetic construct
  source 1..20: mol_type = other RNA
cccagaccgccagtgactgg

SEQ ID NO: 13250 - RNA, 20 nt, synthetic construct
  source 1..20: mol_type = other RNA
gtcactggcggtctgggaga

SEQ ID NO: 13251 - RNA, 20 nt, synthetic construct
  source 1..20: mol_type = other RNA
ctcccagaccgccagtgact

SEQ ID NO: 13252 - RNA, 20 nt, synthetic construct
  source 1..20: mol_type = other RNA
tctcccagaccgccagtgac

SEQ ID NO: 13253 - RNA, 20 nt, synthetic construct
  source 1..20: mol_type = other RNA
tgaagccccaacccccacag

SEQ ID NO: 13254 - RNA, 20 nt, synthetic construct
  source 1..20: mol_type = other RNA
gaagccccaacccccacagc

SEQ ID NO: 13255 - RNA, 20 nt, synthetic construct
  source 1..20: mol_type = other RNA
aagccccaacccccacagcg

SEQ ID NO: 13256 - RNA, 20 nt, synthetic construct
  source 1..20: mol_type = other RNA
gctgtgggggttggggcttc

SEQ ID NO: 13257 - RNA, 20 nt, synthetic construct
  source 1..20: mol_type = other RNA
ccccaacccccacagcgggg

SEQ ID NO: 13258 - RNA, 20 nt, synthetic construct
  source 1..20: mol_type = other RNA
cctccccgctgtgggggttg

SEQ ID NO: 13259 - RNA, 20 nt, synthetic construct
  source 1..20: mol_type = other RNA
cccccacagcggggaggtca

SEQ ID NO: 13260 - RNA, 20 nt, synthetic construct
  source 1..20: mol_type = other RNA
gacctccccgctgtgggggt

SEQ ID NO: 13261 - RNA, 20 nt, synthetic construct
  source 1..20: mol_type = other RNA
ccctgacctccccgctgtgg

SEQ ID NO: 13262 - RNA, 20 nt, synthetic construct
  source 1..20: mol_type = other RNA
cccctgacctccccgctgtg

SEQ ID NO: 13263 - RNA, 20 nt, synthetic construct
  source 1..20: mol_type = other RNA
gcccctgacctccccgctgt

SEQ ID NO: 13264 - RNA, 20 nt, synthetic construct
  source 1..20: mol_type = other RNA
ggcccctgacctccccgctg

SEQ ID NO: 13265 - RNA, 20 nt, synthetic construct
  source 1..20: mol_type = other RNA
ggaggtcaggggccctggtc

SEQ ID NO: 13266 - RNA, 20 nt, synthetic construct
  source 1..20: mol_type = other RNA
gtcaggggccctggtcaggc

SEQ ID NO: 13267 - RNA, 20 nt, synthetic construct
  source 1..20: mol_type = other RNA
tcaggggccctggtcaggct

SEQ ID NO: 13268 - RNA, 20 nt, synthetic construct
  source 1..20: mol_type = other RNA
caggggccctggtcaggctg

SEQ ID NO: 13269 - RNA, 20 nt, synthetic construct
  source 1..20: mol_type = other RNA
ctggtcaggctggggacttc

SEQ ID NO: 13270 - RNA, 20 nt, synthetic construct
  source 1..20: mol_type = other RNA
tgaagtccccagcctgacca

SEQ ID NO: 13271 - RNA, 20 nt, synthetic construct
  source 1..20: mol_type = other RNA
ctgaagtccccagcctgacc

SEQ ID NO: 13272 - RNA, 20 nt, synthetic construct
  source 1..20: mol_type = other RNA
acttcaggccccctttgccc

SEQ ID NO: 13273 - RNA, 20 nt, synthetic construct
  source 1..20: mol_type = other RNA
ccccctttgccctggccccc

SEQ ID NO: 13274 - RNA, 20 nt, synthetic construct
  source 1..20: mol_type = other RNA
cctgggggccagggcaaagg

SEQ ID NO: 13275 - RNA, 20 nt, synthetic construct
  source 1..20: mol_type = other RNA
tcctgggggccagggcaaag

SEQ ID NO: 13276 - RNA, 20 nt, synthetic construct
  source 1..20: mol_type = other RNA
ttcctgggggccagggcaaa

SEQ ID NO: 13277 - RNA, 20 nt, synthetic construct
  source 1..20: mol_type = other RNA
gttcctgggggccagggcaa

SEQ ID NO: 13278 - RNA, 20 nt, synthetic construct
  source 1..20: mol_type = other RNA
gatgaggttcctgggggcca

SEQ ID NO: 13279 - RNA, 20 nt, synthetic construct
  source 1..20: mol_type = other RNA
ggatgaggttcctgggggcc

SEQ ID NO: 13280 - RNA, 20 nt, synthetic construct
  source 1..20: mol_type = other RNA
agcgaggatgaggttcctgg

SEQ ID NO: 13281 - RNA, 20 nt, synthetic construct
  source 1..20: mol_type = other RNA
tagcgaggatgaggttcctg

SEQ ID NO: 13282 - RNA, 20 nt, synthetic construct
  source 1..20: mol_type = other RNA
ctagcgaggatgaggttcct

SEQ ID NO: 13283 - RNA, 20 nt, synthetic construct
  source 1..20: mol_type = other RNA
tctagcgaggatgaggttcc

SEQ ID NO: 13284 - RNA, 20 nt, synthetic construct
  source 1..20: mol_type = other RNA
ctcatcctcgctagaggcat

SEQ ID NO: 13285 - RNA, 20 nt, synthetic construct
  source 1..20: mol_type = other RNA
tcatcctcgctagaggcatt

SEQ ID NO: 13286 - RNA, 20 nt, synthetic construct
  source 1..20: mol_type = other RNA
catcctcgctagaggcattg

SEQ ID NO: 13287 - RNA, 20 nt, synthetic construct
  source 1..20: mol_type = other RNA
caatgcctctagcgaggatg

SEQ ID NO: 13288 - RNA, 20 nt, synthetic construct
  source 1..20: mol_type = other RNA
cctcgctagaggcattgggg

SEQ ID NO: 13289 - RNA, 20 nt, synthetic construct
  source 1..20: mol_type = other RNA
ctcgctagaggcattggggt

SEQ ID NO: 13290 - RNA, 20 nt, synthetic construct
  source 1..20: mol_type = other RNA
tcgctagaggcattggggtg

SEQ ID NO: 13291 - RNA, 20 nt, synthetic construct
  source 1..20: mol_type = other RNA
ccaccccaatgcctctagcg

SEQ ID NO: 13292 - RNA, 20 nt, synthetic construct
  source 1..20: mol_type = other RNA
gaggcattggggtggggacc

SEQ ID NO: 13293 - RNA, 20 nt, synthetic construct
  source 1..20: mol_type = other RNA
ggggtggggaccaggctgcg

SEQ ID NO: 13294 - RNA, 20 nt, synthetic construct
  source 1..20: mol_type = other RNA
gaggatgactcctcgcagcc

SEQ ID NO: 13295 - RNA, 20 nt, synthetic construct
  source 1..20: mol_type = other RNA
gagtcatcctcaaacatttc

SEQ ID NO: 13296 - RNA, 20 nt, synthetic construct
  source 1..20: mol_type = other RNA
agtcatcctcaaacatttca

SEQ ID NO: 13297 - RNA, 20 nt, synthetic construct
  source 1..20: mol_type = other RNA
ggagaaccctgaaatgtttg

SEQ ID NO: 13298 - RNA, 20 nt, synthetic construct
  source 1..20: mol_type = other RNA
cagggttctccagcatctct

SEQ ID NO: 13299 - RNA, 20 nt, synthetic construct
  source 1..20: mol_type = other RNA
ctccagcatctctcggatta

SEQ ID NO: 13300 - RNA, 20 nt, synthetic construct
  source 1..20: mol_type = other RNA
tccagcatctctcggattaa

SEQ ID NO: 13301 - RNA, 20 nt, synthetic construct
  source 1..20: mol_type = other RNA
agcatctctcggattaaggg

SEQ ID NO: 13302 - RNA, 20 nt, synthetic construct
  source 1..20: mol_type = other RNA
tcccttaatccgagagatgc

SEQ ID NO: 13303 - RNA, 20 nt, synthetic construct
  source 1..20: mol_type = other RNA
tctcggattaagggaggcat

SEQ ID NO: 13304 - RNA, 20 nt, synthetic construct
  source 1..20: mol_type = other RNA
ctcggattaagggaggcatc

SEQ ID NO: 13305 - RNA, 20 nt, synthetic construct
  source 1..20: mol_type = other RNA
attaagggaggcatcgggcc

SEQ ID NO: 13306 - RNA, 20 nt, synthetic construct
  source 1..20: mol_type = other RNA
aatctccatcttcagagtaa

SEQ ID NO: 13307 - RNA, 20 nt, synthetic construct
  source 1..20: mol_type = other RNA
aagggccattactctgaaga

SEQ ID NO: 13308 - RNA, 20 nt, synthetic construct
  source 1..20: mol_type = other RNA
ggccctttcagctcctacaa

SEQ ID NO: 13309 - RNA, 20 nt, synthetic construct
  source 1..20: mol_type = other RNA
ctccattgtaggagctgaaa

SEQ ID NO: 13310 - RNA, 20 nt, synthetic construct
  source 1..20: mol_type = other RNA
tctccattgtaggagctgaa

SEQ ID NO: 13311 - RNA, 20 nt, synthetic construct
  source 1..20: mol_type = other RNA
caatggagagagaaagagag

SEQ ID NO: 13312 - RNA, 20 nt, synthetic construct
  source 1..20: mol_type = other RNA
tctctttctctctccattgt

SEQ ID NO: 13313 - RNA, 20 nt, synthetic construct
  source 1..20: mol_type = other RNA
agagagaaagagagaggctc

SEQ ID NO: 13314 - RNA, 20 nt, synthetic construct
  source 1..20: mol_type = other RNA
gagaaagagagaggctcagg

SEQ ID NO: 13315 - RNA, 20 nt, synthetic construct
  source 1..20: mol_type = other RNA
agagaggctcaggaggacag

SEQ ID NO: 13316 - RNA, 20 nt, synthetic construct
  source 1..20: mol_type = other RNA
ctcaggaggacagaggcaca

SEQ ID NO: 13317 - RNA, 20 nt, synthetic construct
  source 1..20: mol_type = other RNA
acagaggcacatggccctta

SEQ ID NO: 13318 - RNA, 20 nt, synthetic construct
  source 1..20: mol_type = other RNA
ggttagggagatggccttaa

SEQ ID NO: 13319 - RNA, 20 nt, synthetic construct
  source 1..20: mol_type = other RNA
aggttagggagatggcctta

SEQ ID NO: 13320 - RNA, 20 nt, synthetic construct
  source 1..20: mol_type = other RNA
gttgagaaaggttagggaga

SEQ ID NO: 13321 - RNA, 20 nt, synthetic construct
  source 1..20: mol_type = other RNA
ggggcagttgagaaaggtta

SEQ ID NO: 13322 - RNA, 20 nt, synthetic construct
  source 1..20: mol_type = other RNA
aggggcagttgagaaaggtt

SEQ ID NO: 13323 - RNA, 20 nt, synthetic construct
  source 1..20: mol_type = other RNA
gagtcaggggcagttgagaa

SEQ ID NO: 13324 - RNA, 20 nt, synthetic construct
  source 1..20: mol_type = other RNA
caactgcccctgactcccct

SEQ ID NO: 13325 - RNA, 20 nt, synthetic construct
  source 1..20: mol_type = other RNA
aactgcccctgactccccta

SEQ ID NO: 13326 - RNA, 20 nt, synthetic construct
  source 1..20: mol_type = other RNA
actgcccctgactcccctag

SEQ ID NO: 13327 - RNA, 20 nt, synthetic construct
  source 1..20: mol_type = other RNA
ctgcccctgactcccctagg

SEQ ID NO: 13328 - RNA, 20 nt, synthetic construct
  source 1..20: mol_type = other RNA
gcgccccctaggggagtcag

SEQ ID NO: 13329 - RNA, 20 nt, synthetic construct
  source 1..20: mol_type = other RNA
ggcgccccctaggggagtca

SEQ ID NO: 13330 - RNA, 20 nt, synthetic construct
  source 1..20: mol_type = other RNA
gggcgccccctaggggagtc

SEQ ID NO: 13331 - RNA, 20 nt, synthetic construct
  source 1..20: mol_type = other RNA
ccctagggggcgcccagcac

SEQ ID NO: 13332 - RNA, 20 nt, synthetic construct
  source 1..20: mol_type = other RNA
ctgtgctgggcgccccctag

SEQ ID NO: 13333 - RNA, 20 nt, synthetic construct
  source 1..20: mol_type = other RNA
cctgtgctgggcgcccccta

SEQ ID NO: 13334 - RNA, 20 nt, synthetic construct
  source 1..20: mol_type = other RNA
gcctgtgctgggcgccccct

SEQ ID NO: 13335 - RNA, 20 nt, synthetic construct
  source 1..20: mol_type = other RNA
gagaaccaggcaatctacac

SEQ ID NO: 13336 - RNA, 20 nt, synthetic construct
  source 1..20: mol_type = other RNA
gaacagagtagttgagaacc

SEQ ID NO: 13337 - RNA, 20 nt, synthetic construct
  source 1..20: mol_type = other RNA
gtgtgtcctcctgtccgacc

SEQ ID NO: 13338 - RNA, 20 nt, synthetic construct
  source 1..20: mol_type = other RNA
tgtgtcctcctgtccgacct

SEQ ID NO: 13339 - RNA, 20 nt, synthetic construct
  source 1..20: mol_type = other RNA
ggtctcccaggtcggacagg

SEQ ID NO: 13340 - RNA, 20 nt, synthetic construct
  source 1..20: mol_type = other RNA
gttggtctcccaggtcggac

SEQ ID NO: 13341 - RNA, 20 nt, synthetic construct
  source 1..20: mol_type = other RNA
acctgggagaccaacagccc

SEQ ID NO: 13342 - RNA, 20 nt, synthetic construct
  source 1..20: mol_type = other RNA
cctgggagaccaacagccct

SEQ ID NO: 13343 - RNA, 20 nt, synthetic construct
  source 1..20: mol_type = other RNA
gggctgttggtctcccaggt

SEQ ID NO: 13344 - RNA, 20 nt, synthetic construct
  source 1..20: mol_type = other RNA
cccagggctgttggtctccc

SEQ ID NO: 13345 - RNA, 20 nt, synthetic construct
  source 1..20: mol_type = other RNA
acagccctgggaagacagag

SEQ ID NO: 13346 - RNA, 20 nt, synthetic construct
  source 1..20: mol_type = other RNA
cagccctgggaagacagaga

SEQ ID NO: 13347 - RNA, 20 nt, synthetic construct
  source 1..20: mol_type = other RNA
agccctgggaagacagagag

SEQ ID NO: 13348 - RNA, 20 nt, synthetic construct
  source 1..20: mol_type = other RNA
gtcccctctctgtcttccca

SEQ ID NO: 13349 - RNA, 20 nt, synthetic construct
  source 1..20: mol_type = other RNA
tgtcccctctctgtcttccc

SEQ ID NO: 13350 - RNA, 20 nt, synthetic construct
  source 1..20: mol_type = other RNA
actaagggtgagtcatgagt

SEQ ID NO: 13351 - RNA, 20 nt, synthetic construct
  source 1..20: mol_type = other RNA
cactaagggtgagtcatgag

SEQ ID NO: 13352 - RNA, 20 nt, synthetic construct
  source 1..20: mol_type = other RNA
cacccttagtgctgatgccc

SEQ ID NO: 13353 - RNA, 20 nt, synthetic construct
  source 1..20: mol_type = other RNA
ccttagtgctgatgccccgg

SEQ ID NO: 13354 - RNA, 20 nt, synthetic construct
  source 1..20: mol_type = other RNA
agtgctgatgccccggaggt

SEQ ID NO: 13355 - RNA, 20 nt, synthetic construct
  source 1..20: mol_type = other RNA
cctccggggcatcagcacta

SEQ ID NO: 13356 - RNA, 20 nt, synthetic construct
  source 1..20: mol_type = other RNA
atgaaaatcaccgacctccg

SEQ ID NO: 13357 - RNA, 20 nt, synthetic construct
  source 1..20: mol_type = other RNA
aatgaaaatcaccgacctcc

SEQ ID NO: 13358 - RNA, 20 nt, synthetic construct
  source 1..20: mol_type = other RNA
taatgaaaatcaccgacctc

SEQ ID NO: 13359 - RNA, 20 nt, synthetic construct
  source 1..20: mol_type = other RNA
gtgattttcattagcatcct

SEQ ID NO: 13360 - RNA, 20 nt, synthetic construct
  source 1..20: mol_type = other RNA
tgattttcattagcatcctt

SEQ ID NO: 13361 - RNA, 20 nt, synthetic construct
  source 1..20: mol_type = other RNA
tagcatccttgggaacatgt

SEQ ID NO: 13362 - RNA, 20 nt, synthetic construct
  source 1..20: mol_type = other RNA
agcatccttgggaacatgta

SEQ ID NO: 13363 - RNA, 20 nt, synthetic construct
  source 1..20: mol_type = other RNA
tccttgggaacatgtagggc

SEQ ID NO: 13364 - RNA, 20 nt, synthetic construct
  source 1..20: mol_type = other RNA
tgggaacatgtagggctggc

SEQ ID NO: 13365 - RNA, 20 nt, synthetic construct
  source 1..20: mol_type = other RNA
gggaacatgtagggctggct

SEQ ID NO: 13366 - RNA, 20 nt, synthetic construct
  source 1..20: mol_type = other RNA
gccagccctacatgttccca

SEQ ID NO: 13367 - RNA, 20 nt, synthetic construct
  source 1..20: mol_type = other RNA
tgtagggctggctgggccgc

SEQ ID NO: 13368 - RNA, 20 nt, synthetic construct
  source 1..20: mol_type = other RNA
gctggctgggccgccggcgc

SEQ ID NO: 13369 - RNA, 20 nt, synthetic construct
  source 1..20: mol_type = other RNA
ctggctgggccgccggcgcc

SEQ ID NO: 13370 - RNA, 20 nt, synthetic construct
  source 1..20: mol_type = other RNA
ggctgtacgcccggcgccgg

SEQ ID NO: 13371 - RNA, 20 nt, synthetic construct
  source 1..20: mol_type = other RNA
gcgccgggcgtacagcctca

SEQ ID NO: 13372 - RNA, 20 nt, synthetic construct
  source 1..20: mol_type = other RNA
tgaggctgtacgcccggcgc

SEQ ID NO: 13373 - RNA, 20 nt, synthetic construct
  source 1..20: mol_type = other RNA
aagccctgaggctgtacgcc

SEQ ID NO: 13374 - RNA, 20 nt, synthetic construct
  source 1..20: mol_type = other RNA
agcctcagggcttccagcag

SEQ ID NO: 13375 - RNA, 20 nt, synthetic construct
  source 1..20: mol_type = other RNA
agccactgctggaagccctg

SEQ ID NO: 13376 - RNA, 20 nt, synthetic construct
  source 1..20: mol_type = other RNA
caagctgcaggagccactgc

SEQ ID NO: 13377 - RNA, 20 nt, synthetic construct
  source 1..20: mol_type = other RNA
ctgcagcttgtccacttttt

SEQ ID NO: 13378 - RNA, 20 nt, synthetic construct
  source 1..20: mol_type = other RNA
tgcagcttgtccactttttc

SEQ ID NO: 13379 - RNA, 20 nt, synthetic construct
  source 1..20: mol_type = other RNA
cgaaaaagtggacaagctgc

SEQ ID NO: 13380 - RNA, 20 nt, synthetic construct
  source 1..20: mol_type = other RNA
ccactttttcgggctcctcc

SEQ ID NO: 13381 - RNA, 20 nt, synthetic construct
  source 1..20: mol_type = other RNA
cctggaggagcccgaaaaag

SEQ ID NO: 13382 - RNA, 20 nt, synthetic construct
  source 1..20: mol_type = other RNA
cgggctcctccaggtccatg

SEQ ID NO: 13383 - RNA, 20 nt, synthetic construct
  source 1..20: mol_type = other RNA
ctccaggtccatgcggtcta

SEQ ID NO: 13384 - RNA, 20 nt, synthetic construct
  source 1..20: mol_type = other RNA
tccaggtccatgcggtctat

SEQ ID NO: 13385 - RNA, 20 nt, synthetic construct
  source 1..20: mol_type = other RNA
ccaggtccatgcggtctatg

SEQ ID NO: 13386 - RNA, 20 nt, synthetic construct
  source 1..20: mol_type = other RNA
catagaccgcatggacctgg

SEQ ID NO: 13387 - RNA, 20 nt, synthetic construct
  source 1..20: mol_type = other RNA
ccccatagaccgcatggacc

SEQ ID NO: 13388 - RNA, 20 nt, synthetic construct
  source 1..20: mol_type = other RNA
acttgtccccatagaccgca

SEQ ID NO: 13389 - RNA, 20 nt, synthetic construct
  source 1..20: mol_type = other RNA
gtctatggggacaagtatac

SEQ ID NO: 13390 - RNA, 20 nt, synthetic construct
  source 1..20: mol_type = other RNA
gacaagtatactggagtgag

SEQ ID NO: 13391 - RNA, 20 nt, synthetic construct
  source 1..20: mol_type = other RNA
acaagtatactggagtgaga

SEQ ID NO: 13392 - RNA, 20 nt, synthetic construct
  source 1..20: mol_type = other RNA
caagtatactggagtgagag

SEQ ID NO: 13393 - RNA, 20 nt, synthetic construct
  source 1..20: mol_type = other RNA
tatactggagtgagagggga

SEQ ID NO: 13394 - RNA, 20 nt, synthetic construct
  source 1..20: mol_type = other RNA
gtgagaggggaaggaagaga

SEQ ID NO: 13395 - RNA, 20 nt, synthetic construct
  source 1..20: mol_type = other RNA
tgagaggggaaggaagagat

SEQ ID NO: 13396 - RNA, 20 nt, synthetic construct
  source 1..20: mol_type = other RNA
gagaggggaaggaagagatg

SEQ ID NO: 13397 - RNA, 20 nt, synthetic construct
  source 1..20: mol_type = other RNA
ggggaagacacagtgacaga

SEQ ID NO: 13398 - RNA, 20 nt, synthetic construct
  source 1..20: mol_type = other RNA
acagatggctgatcaccaac

SEQ ID NO: 13399 - RNA, 20 nt, synthetic construct
  source 1..20: mol_type = other RNA
ctgatcaccaaccggcgttt

SEQ ID NO: 13400 - RNA, 20 nt, synthetic construct
  source 1..20: mol_type = other RNA
tgatcaccaaccggcgtttt

SEQ ID NO: 13401 - RNA, 20 nt, synthetic construct
  source 1..20: mol_type = other RNA
aggcttcccaaaacgccggt

SEQ ID NO: 13402 - RNA, 20 nt, synthetic construct
  source 1..20: mol_type = other RNA
gcgttttgggaagcctgtac

SEQ ID NO: 13403 - RNA, 20 nt, synthetic construct
  source 1..20: mol_type = other RNA
cgttttgggaagcctgtaca

SEQ ID NO: 13404 - RNA, 20 nt, synthetic construct
  source 1..20: mol_type = other RNA
gtacaggcttcccaaaacgc

SEQ ID NO: 13405 - RNA, 20 nt, synthetic construct
  source 1..20: mol_type = other RNA
tacagggtttcagaactctc

SEQ ID NO: 13406 - RNA, 20 nt, synthetic construct
  source 1..20: mol_type = other RNA
agagttctgaaaccctgtac

SEQ ID NO: 13407 - RNA, 20 nt, synthetic construct
  source 1..20: mol_type = other RNA
gggtttcagaactctctgga

SEQ ID NO: 13408 - RNA, 20 nt, synthetic construct
  source 1..20: mol_type = other RNA
ggtttcagaactctctggat

SEQ ID NO: 13409 - RNA, 20 nt, synthetic construct
  source 1..20: mol_type = other RNA
gtttcagaactctctggatg

SEQ ID NO: 13410 - RNA, 20 nt, synthetic construct
  source 1..20: mol_type = other RNA
ctgctggtaattcttgcacc

SEQ ID NO: 13411 - RNA, 20 nt, synthetic construct
  source 1..20: mol_type = other RNA
ttaccagcagaagagaccac

SEQ ID NO: 13412 - RNA, 20 nt, synthetic construct
  source 1..20: mol_type = other RNA
taccagcagaagagaccact

SEQ ID NO: 13413 - RNA, 20 nt, synthetic construct
  source 1..20: mol_type = other RNA
gacccagtggtctcttctgc

SEQ ID NO: 13414 - RNA, 20 nt, synthetic construct
  source 1..20: mol_type = other RNA
agggggcgtggaggacccag

SEQ ID NO: 13415 - RNA, 20 nt, synthetic construct
  source 1..20: mol_type = other RNA
ctgtctgggagggggcgtgg

SEQ ID NO: 13416 - RNA, 20 nt, synthetic construct
  source 1..20: mol_type = other RNA
aatctgtctgggagggggcg

SEQ ID NO: 13417 - RNA, 20 nt, synthetic construct
  source 1..20: mol_type = other RNA
cctcccagacagattccgca

SEQ ID NO: 13418 - RNA, 20 nt, synthetic construct
  source 1..20: mol_type = other RNA
tgcggaatctgtctgggagg

SEQ ID NO: 13419 - RNA, 20 nt, synthetic construct
  source 1..20: mol_type = other RNA
atgcggaatctgtctgggag

SEQ ID NO: 13420 - RNA, 20 nt, synthetic construct
  source 1..20: mol_type = other RNA
catgcggaatctgtctggga

SEQ ID NO: 13421 - RNA, 20 nt, synthetic construct
  source 1..20: mol_type = other RNA
cagacagattccgcatggag

SEQ ID NO: 13422 - RNA, 20 nt, synthetic construct
  source 1..20: mol_type = other RNA
actccatgcggaatctgtct

SEQ ID NO: 13423 - RNA, 20 nt, synthetic construct
  source 1..20: mol_type = other RNA
cagattccgcatggagtggt

SEQ ID NO: 13424 - RNA, 20 nt, synthetic construct
  source 1..20: mol_type = other RNA
tccgcatggagtggtgggaa

SEQ ID NO: 13425 - RNA, 20 nt, synthetic construct
  source 1..20: mol_type = other RNA
tcctttcccaccactccatg

SEQ ID NO: 13426 - RNA, 20 nt, synthetic construct
  source 1..20: mol_type = other RNA
ctgagcactgagcagacgcc

SEQ ID NO: 13427 - RNA, 20 nt, synthetic construct
  source 1..20: mol_type = other RNA
tgagcactgagcagacgcca

SEQ ID NO: 13428 - RNA, 20 nt, synthetic construct
  source 1..20: mol_type = other RNA
gagcactgagcagacgccag

SEQ ID NO: 13429 - RNA, 20 nt, synthetic construct
  source 1..20: mol_type = other RNA
agcactgagcagacgccagg

SEQ ID NO: 13430 - RNA, 20 nt, synthetic construct
  source 1..20: mol_type = other RNA
ggaggtgcgggggcgccccc

SEQ ID NO: 13431 - RNA, 20 nt, synthetic construct
  source 1..20: mol_type = other RNA
cccccgcacctccgcagatg

SEQ ID NO: 13432 - RNA, 20 nt, synthetic construct
  source 1..20: mol_type = other RNA
cctcatctgcggaggtgcgg

SEQ ID NO: 13433 - RNA, 20 nt, synthetic construct
  source 1..20: mol_type = other RNA
gcctcatctgcggaggtgcg

SEQ ID NO: 13434 - RNA, 20 nt, synthetic construct
  source 1..20: mol_type = other RNA
tgcctcatctgcggaggtgc

SEQ ID NO: 13435 - RNA, 20 nt, synthetic construct
  source 1..20: mol_type = other RNA
ctgcctcatctgcggaggtg

SEQ ID NO: 13436 - RNA, 20 nt, synthetic construct
  source 1..20: mol_type = other RNA
gccatctgcctcatctgcgg

SEQ ID NO: 13437 - RNA, 20 nt, synthetic construct
  source 1..20: mol_type = other RNA
agcgccatctgcctcatctg

SEQ ID NO: 13438 - RNA, 20 nt, synthetic construct
  source 1..20: mol_type = other RNA
ggcgctgagcagccctgtct

SEQ ID NO: 13439 - RNA, 20 nt, synthetic construct
  source 1..20: mol_type = other RNA
agatggatgacaccgagaca

SEQ ID NO: 13440 - RNA, 20 nt, synthetic construct
  source 1..20: mol_type = other RNA
gagatggatgacaccgagac

SEQ ID NO: 13441 - RNA, 20 nt, synthetic construct
  source 1..20: mol_type = other RNA
tcggtgtcatccatctccag

SEQ ID NO: 13442 - RNA, 20 nt, synthetic construct
  source 1..20: mol_type = other RNA
tgtcatccatctccaggggc

SEQ ID NO: 13443 - RNA, 20 nt, synthetic construct
  source 1..20: mol_type = other RNA
gcagctcctgcccctggaga

SEQ ID NO: 13444 - RNA, 20 nt, synthetic construct
  source 1..20: mol_type = other RNA
gggcaggagctgcccagcaa

SEQ ID NO: 13445 - RNA, 20 nt, synthetic construct
  source 1..20: mol_type = other RNA
tgctgggcagctcctgcccc

SEQ ID NO: 13446 - RNA, 20 nt, synthetic construct
  source 1..20: mol_type = other RNA
gcccagcaaaggcaaagaca

SEQ ID NO: 13447 - RNA, 20 nt, synthetic construct
  source 1..20: mol_type = other RNA
accttgtctttgcctttgct

SEQ ID NO: 13448 - RNA, 20 nt, synthetic construct
  source 1..20: mol_type = other RNA
gaccttgtctttgcctttgc

SEQ ID NO: 13449 - RNA, 20 nt, synthetic construct
  source 1..20: mol_type = other RNA
aggcaaagacaaggtctgtg

SEQ ID NO: 13450 - RNA, 20 nt, synthetic construct
  source 1..20: mol_type = other RNA
ggcaaagacaaggtctgtga

SEQ ID NO: 13451 - RNA, 20 nt, synthetic construct
  source 1..20: mol_type = other RNA
gcaaagacaaggtctgtgag

SEQ ID NO: 13452 - RNA, 20 nt, synthetic construct
  source 1..20: mol_type = other RNA
gtctgtgaggggcccgaagc

SEQ ID NO: 13453 - RNA, 20 nt, synthetic construct
  source 1..20: mol_type = other RNA
cgaagccggcattgtgcatc

SEQ ID NO: 13454 - RNA, 20 nt, synthetic construct
  source 1..20: mol_type = other RNA
gaagccggcattgtgcatct

SEQ ID NO: 13455 - RNA, 20 nt, synthetic construct
  source 1..20: mol_type = other RNA
agatgcacaatgccggcttc

SEQ ID NO: 13456 - RNA, 20 nt, synthetic construct
  source 1..20: mol_type = other RNA
cagatgcacaatgccggctt

SEQ ID NO: 13457 - RNA, 20 nt, synthetic construct
  source 1..20: mol_type = other RNA
cggcattgtgcatctgggtc

SEQ ID NO: 13458 - RNA, 20 nt, synthetic construct
  source 1..20: mol_type = other RNA
cggacccagatgcacaatgc

SEQ ID NO: 13459 - RNA, 20 nt, synthetic construct
  source 1..20: mol_type = other RNA
tgtgcatctgggtccggttc

SEQ ID NO: 13460 - RNA, 20 nt, synthetic construct
  source 1..20: mol_type = other RNA
gtgcatctgggtccggttca

SEQ ID NO: 13461 - RNA, 20 nt, synthetic construct
  source 1..20: mol_type = other RNA
ccggttcagggtcagcccgt

SEQ ID NO: 13462 - RNA, 20 nt, synthetic construct
  source 1..20: mol_type = other RNA
ccgacgggctgaccctgaac

SEQ ID NO: 13463 - RNA, 20 nt, synthetic construct
  source 1..20: mol_type = other RNA
cagggtcagcccgtcggaga

SEQ ID NO: 13464 - RNA, 20 nt, synthetic construct
  source 1..20: mol_type = other RNA
cagcccgtcggagaaggtca

SEQ ID NO: 13465 - RNA, 20 nt, synthetic construct
  source 1..20: mol_type = other RNA
acaccatgaccttctccgac

SEQ ID NO: 13466 - RNA, 20 nt, synthetic construct
  source 1..20: mol_type = other RNA
gacaccatgaccttctccga

SEQ ID NO: 13467 - RNA, 20 nt, synthetic construct
  source 1..20: mol_type = other RNA
aaggtcatggtgtcctgctc

SEQ ID NO: 13468 - RNA, 20 nt, synthetic construct
  source 1..20: mol_type = other RNA
aggtcatggtgtcctgctct

SEQ ID NO: 13469 - RNA, 20 nt, synthetic construct
  source 1..20: mol_type = other RNA
ggtcatggtgtcctgctctg

SEQ ID NO: 13470 - RNA, 20 nt, synthetic construct
  source 1..20: mol_type = other RNA
cacaaggtacaccccagagc

SEQ ID NO: 13471 - RNA, 20 nt, synthetic construct
  source 1..20: mol_type = other RNA
ttgtgcagatacgcagcatc

SEQ ID NO: 13472 - RNA, 20 nt, synthetic construct
  source 1..20: mol_type = other RNA
agatgctgcgtatctgcaca

SEQ ID NO: 13473 - RNA, 20 nt, synthetic construct
  source 1..20: mol_type = other RNA
agatacgcagcatctggagg

SEQ ID NO: 13474 - RNA, 20 nt, synthetic construct
  source 1..20: mol_type = other RNA
gatacgcagcatctggaggt

SEQ ID NO: 13475 - RNA, 20 nt, synthetic construct
  source 1..20: mol_type = other RNA
atacgcagcatctggaggtg

SEQ ID NO: 13476 - RNA, 20 nt, synthetic construct
  source 1..20: mol_type = other RNA
tacgcagcatctggaggtgg

SEQ ID NO: 13477 - RNA, 20 nt, synthetic construct
  source 1..20: mol_type = other RNA
acgcagcatctggaggtggg

SEQ ID NO: 13478 - RNA, 20 nt, synthetic construct
  source 1..20: mol_type = other RNA
cagcatctggaggtgggggg

SEQ ID NO: 13479 - RNA, 20 nt, synthetic construct
  source 1..20: mol_type = other RNA
catctggaggtggggggtgg

SEQ ID NO: 13480 - RNA, 20 nt, synthetic construct
  source 1..20: mol_type = other RNA
ctggaggtggggggtggagg

SEQ ID NO: 13481 - RNA, 20 nt, synthetic construct
  source 1..20: mol_type = other RNA
tggaggtggggggtggagga

SEQ ID NO: 13482 - RNA, 20 nt, synthetic construct
  source 1..20: mol_type = other RNA
aggagggttagtgctgtttc

SEQ ID NO: 13483 - RNA, 20 nt, synthetic construct
  source 1..20: mol_type = other RNA
ggagggttagtgctgtttct

SEQ ID NO: 13484 - RNA, 20 nt, synthetic construct
  source 1..20: mol_type = other RNA
gagggttagtgctgtttctg

SEQ ID NO: 13485 - RNA, 20 nt, synthetic construct
  source 1..20: mol_type = other RNA
agggttagtgctgtttctgg

SEQ ID NO: 13486 - RNA, 20 nt, synthetic construct
  source 1..20: mol_type = other RNA
ttagtgctgtttctggggga

SEQ ID NO: 13487 - RNA, 20 nt, synthetic construct
  source 1..20: mol_type = other RNA
tagtgctgtttctgggggat

SEQ ID NO: 13488 - RNA, 20 nt, synthetic construct
  source 1..20: mol_type = other RNA
agtgctgtttctgggggatg

SEQ ID NO: 13489 - RNA, 20 nt, synthetic construct
  source 1..20: mol_type = other RNA
ttctgggggatggggaaaag

SEQ ID NO: 13490 - RNA, 20 nt, synthetic construct
  source 1..20: mol_type = other RNA
tctgggggatggggaaaaga

SEQ ID NO: 13491 - RNA, 20 nt, synthetic construct
  source 1..20: mol_type = other RNA
tggggaaaagagggaatgag

SEQ ID NO: 13492 - RNA, 20 nt, synthetic construct
  source 1..20: mol_type = other RNA
gagggaatgagtggaaagtg

SEQ ID NO: 13493 - RNA, 20 nt, synthetic construct
  source 1..20: mol_type = other RNA
ggaatgagtggaaagtgagg

SEQ ID NO: 13494 - RNA, 20 nt, synthetic construct
  source 1..20: mol_type = other RNA
gagtggaaagtgaggaggtt

SEQ ID NO: 13495 - RNA, 20 nt, synthetic construct
  source 1..20: mol_type = other RNA
cagtgagtgcaacctgaagc

SEQ ID NO: 13496 - RNA, 20 nt, synthetic construct
  source 1..20: mol_type = other RNA
gcttcaggttgcactcactg

SEQ ID NO: 13497 - RNA, 20 nt, synthetic construct
  source 1..20: mol_type = other RNA
tgcttcaggttgcactcact

SEQ ID NO: 13498 - RNA, 20 nt, synthetic construct
  source 1..20: mol_type = other RNA
ctgcttcaggttgcactcac

SEQ ID NO: 13499 - RNA, 20 nt, synthetic construct
  source 1..20: mol_type = other RNA
agtgcaacctgaagcaggca

SEQ ID NO: 13500 - RNA, 20 nt, synthetic construct
  source 1..20: mol_type = other RNA
acctgaagcaggcatggaga

SEQ ID NO: 13501 - RNA, 20 nt, synthetic construct
  source 1..20: mol_type = other RNA
aggagtcccacatgtgtggc

SEQ ID NO: 13502 - RNA, 20 nt, synthetic construct
  source 1..20: mol_type = other RNA
ggagtcccacatgtgtggca

SEQ ID NO: 13503 - RNA, 20 nt, synthetic construct
  source 1..20: mol_type = other RNA
gagtcccacatgtgtggcag

SEQ ID NO: 13504 - RNA, 20 nt, synthetic construct
  source 1..20: mol_type = other RNA
agtcccacatgtgtggcagg

SEQ ID NO: 13505 - RNA, 20 nt, synthetic construct
  source 1..20: mol_type = other RNA
acatgtgtggcagggggtgc

SEQ ID NO: 13506 - RNA, 20 nt, synthetic construct
  source 1..20: mol_type = other RNA
catgtgtggcagggggtgca

SEQ ID NO: 13507 - RNA, 20 nt, synthetic construct
  source 1..20: mol_type = other RNA
gcaccccctgccacacatgt

SEQ ID NO: 13508 - RNA, 20 nt, synthetic construct
  source 1..20: mol_type = other RNA
tgcaccccctgccacacatg

SEQ ID NO: 13509 - RNA, 20 nt, synthetic construct
  source 1..20: mol_type = other RNA
gtggcagggggtgcagggta

SEQ ID NO: 13510 - RNA, 20 nt, synthetic construct
  source 1..20: mol_type = other RNA
agggtaaggaaatctttgca

SEQ ID NO: 13511 - RNA, 20 nt, synthetic construct
  source 1..20: mol_type = other RNA
ggaaatctttgcatggatca

SEQ ID NO: 13512 - RNA, 20 nt, synthetic construct
  source 1..20: mol_type = other RNA
catggatcaaggaattgttg

SEQ ID NO: 13513 - RNA, 20 nt, synthetic construct
  source 1..20: mol_type = other RNA
atggatcaaggaattgttga

SEQ ID NO: 13514 - RNA, 20 nt, synthetic construct
  source 1..20: mol_type = other RNA
attgttgagggtcccatatg

SEQ ID NO: 13515 - RNA, 20 nt, synthetic construct
  source 1..20: mol_type = other RNA
ttgttgagggtcccatatgt

SEQ ID NO: 13516 - RNA, 20 nt, synthetic construct
  source 1..20: mol_type = other RNA
tgagggtcccatatgtgggt

SEQ ID NO: 13517 - RNA, 20 nt, synthetic construct
  source 1..20: mol_type = other RNA
gagggtcccatatgtgggtc

SEQ ID NO: 13518 - RNA, 20 nt, synthetic construct
  source 1..20: mol_type = other RNA
cccatatgtgggtcgggctg

SEQ ID NO: 13519 - RNA, 20 nt, synthetic construct
  source 1..20: mol_type = other RNA
tatgtgggtcgggctgtggc

SEQ ID NO: 13520 - RNA, 20 nt, synthetic construct
  source 1..20: mol_type = other RNA
ccacagcccgacccacatat

SEQ ID NO: 13521 - RNA, 20 nt, synthetic construct
  source 1..20: mol_type = other RNA
gccacagcccgacccacata

SEQ ID NO: 13522 - RNA, 20 nt, synthetic construct
  source 1..20: mol_type = other RNA
cgggctgtggcaggacccac

SEQ ID NO: 13523 - RNA, 20 nt, synthetic construct
  source 1..20: mol_type = other RNA
gggctgtggcaggacccaca

SEQ ID NO: 13524 - RNA, 20 nt, synthetic construct
  source 1..20: mol_type = other RNA
cccacagggcctaacttacc

SEQ ID NO: 13525 - RNA, 20 nt, synthetic construct
  source 1..20: mol_type = other RNA
cctggtaagttaggccctgt

SEQ ID NO: 13526 - RNA, 20 nt, synthetic construct
  source 1..20: mol_type = other RNA
tcctggtaagttaggccctg

SEQ ID NO: 13527 - RNA, 20 nt, synthetic construct
  source 1..20: mol_type = other RNA
cctaacttaccaggatatct

SEQ ID NO: 13528 - RNA, 20 nt, synthetic construct
  source 1..20: mol_type = other RNA
acttaccaggatatctaggc

SEQ ID NO: 13529 - RNA, 20 nt, synthetic construct
  source 1..20: mol_type = other RNA
cctagatatcctggtaagtt

SEQ ID NO: 13530 - RNA, 20 nt, synthetic construct
  source 1..20: mol_type = other RNA
agctgcctgcctagatatcc

SEQ ID NO: 13531 - RNA, 20 nt, synthetic construct
  source 1..20: mol_type = other RNA
cagctttgagcagagtgatc

SEQ ID NO: 13532 - RNA, 20 nt, synthetic construct
  source 1..20: mol_type = other RNA
atgctgagccctgtaaagcc

SEQ ID NO: 13533 - RNA, 20 nt, synthetic construct
  source 1..20: mol_type = other RNA
tgtaaagccaggcaaccgct

SEQ ID NO: 13534 - RNA, 20 nt, synthetic construct
  source 1..20: mol_type = other RNA
agcggttgcctggctttaca

SEQ ID NO: 13535 - RNA, 20 nt, synthetic construct
  source 1..20: mol_type = other RNA
aagcggttgcctggctttac

SEQ ID NO: 13536 - RNA, 20 nt, synthetic construct
  source 1..20: mol_type = other RNA
gagtttgccaagcggttgcc

SEQ ID NO: 13537 - RNA, 20 nt, synthetic construct
  source 1..20: mol_type = other RNA
agatcgtggagtttgccaag

SEQ ID NO: 13538 - RNA, 20 nt, synthetic construct
  source 1..20: mol_type = other RNA
cacgatcttgatgatgcact

SEQ ID NO: 13539 - RNA, 20 nt, synthetic construct
  source 1..20: mol_type = other RNA
caagtgcatcatcaagatcg

SEQ ID NO: 13540 - RNA, 20 nt, synthetic construct
  source 1..20: mol_type = other RNA
gtgggacaagttcagtgagc

SEQ ID NO: 13541 - RNA, 20 nt, synthetic construct
  source 1..20: mol_type = other RNA
gcagctggatctggggctgt

SEQ ID NO: 13542 - RNA, 20 nt, synthetic construct
  source 1..20: mol_type = other RNA
tgcagctggatctggggctg

SEQ ID NO: 13543 - RNA, 20 nt, synthetic construct
  source 1..20: mol_type = other RNA
ccagatccagctgcacgcgg

SEQ ID NO: 13544 - RNA, 20 nt, synthetic construct
  source 1..20: mol_type = other RNA
accgcgtgcagctggatctg

SEQ ID NO: 13545 - RNA, 20 nt, synthetic construct
  source 1..20: mol_type = other RNA
caccgcgtgcagctggatct

SEQ ID NO: 13546 - RNA, 20 nt, synthetic construct
  source 1..20: mol_type = other RNA
ccaccgcgtgcagctggatc

SEQ ID NO: 13547 - RNA, 20 nt, synthetic construct
  source 1..20: mol_type = other RNA
ctgcacgcggtggtctgcac

SEQ ID NO: 13548 - RNA, 20 nt, synthetic construct
  source 1..20: mol_type = other RNA
tgcagaccaccgcgtgcagc

SEQ ID NO: 13549 - RNA, 20 nt, synthetic construct
  source 1..20: mol_type = other RNA
tctgcactggagttctgcag

SEQ ID NO: 13550 - RNA, 20 nt, synthetic construct
  source 1..20: mol_type = other RNA
ctgcactggagttctgcaga

SEQ ID NO: 13551 - RNA, 20 nt, synthetic construct
  source 1..20: mol_type = other RNA
tgcactggagttctgcagag

SEQ ID NO: 13552 - RNA, 20 nt, synthetic construct
  source 1..20: mol_type = other RNA
actggagttctgcagagggg

SEQ ID NO: 13553 - RNA, 20 nt, synthetic construct
  source 1..20: mol_type = other RNA
ctggagttctgcagagggga

SEQ ID NO: 13554 - RNA, 20 nt, synthetic construct
  source 1..20: mol_type = other RNA
tggagttctgcagaggggag

SEQ ID NO: 13555 - RNA, 20 nt, synthetic construct
  source 1..20: mol_type = other RNA
ctgcagaggggaggggtaga

SEQ ID NO: 13556 - RNA, 20 nt, synthetic construct
  source 1..20: mol_type = other RNA
agaggggaggggtagaaggt

SEQ ID NO: 13557 - RNA, 20 nt, synthetic construct
  source 1..20: mol_type = other RNA
gggaggggtagaaggttgga

SEQ ID NO: 13558 - RNA, 20 nt, synthetic construct
  source 1..20: mol_type = other RNA
gaaggttggaaggcaagcta

SEQ ID NO: 13559 - RNA, 20 nt, synthetic construct
  source 1..20: mol_type = other RNA
ggcaagctaaggcccacctc

SEQ ID NO: 13560 - RNA, 20 nt, synthetic construct
  source 1..20: mol_type = other RNA
gcaagctaaggcccacctct

SEQ ID NO: 13561 - RNA, 20 nt, synthetic construct
  source 1..20: mol_type = other RNA
caagctaaggcccacctctg

SEQ ID NO: 13562 - RNA, 20 nt, synthetic construct
  source 1..20: mol_type = other RNA
aagctaaggcccacctctgg

SEQ ID NO: 13563 - RNA, 20 nt, synthetic construct
  source 1..20: mol_type = other RNA
agaagacagcccccagaggt

SEQ ID NO: 13564 - RNA, 20 nt, synthetic construct
  source 1..20: mol_type = other RNA
gagaagacagcccccagagg

SEQ ID NO: 13565 - RNA, 20 nt, synthetic construct
  source 1..20: mol_type = other RNA
agagagaagacagcccccag

SEQ ID NO: 13566 - RNA, 20 nt, synthetic construct
  source 1..20: mol_type = other RNA
gaggagagagcttgggatat

SEQ ID NO: 13567 - RNA, 20 nt, synthetic construct
  source 1..20: mol_type = other RNA
gaatgcagaggagagagctt

SEQ ID NO: 13568 - RNA, 20 nt, synthetic construct
  source 1..20: mol_type = other RNA
agaatgcagaggagagagct

SEQ ID NO: 13569 - RNA, 20 nt, synthetic construct
  source 1..20: mol_type = other RNA
aggagggcatcagaatgcag

SEQ ID NO: 13570 - RNA, 20 nt, synthetic construct
  source 1..20: mol_type = other RNA
actggtgctgaggacaagga

SEQ ID NO: 13571 - RNA, 20 nt, synthetic construct
  source 1..20: mol_type = other RNA
gactggtgctgaggacaagg

SEQ ID NO: 13572 - RNA, 20 nt, synthetic construct
  source 1..20: mol_type = other RNA
atcgactggtgctgaggaca

SEQ ID NO: 13573 - RNA, 20 nt, synthetic construct
  source 1..20: mol_type = other RNA
gctatcatcgactggtgctg

SEQ ID NO: 13574 - RNA, 20 nt, synthetic construct
  source 1..20: mol_type = other RNA
tgttggaggctatcatcgac

SEQ ID NO: 13575 - RNA, 20 nt, synthetic construct
  source 1..20: mol_type = other RNA
atggggctgggttgtgttgg

SEQ ID NO: 13576 - RNA, 20 nt, synthetic construct
  source 1..20: mol_type = other RNA
ggaatggggctgggttgtgt

SEQ ID NO: 13577 - RNA, 20 nt, synthetic construct
  source 1..20: mol_type = other RNA
tcactttggggaatggggct

SEQ ID NO: 13578 - RNA, 20 nt, synthetic construct
  source 1..20: mol_type = other RNA
ttcactttggggaatggggc

SEQ ID NO: 13579 - RNA, 20 nt, synthetic construct
  source 1..20: mol_type = other RNA
actcttcactttggggaatg

SEQ ID NO: 13580 - RNA, 20 nt, synthetic construct
  source 1..20: mol_type = other RNA
cactcttcactttggggaat

SEQ ID NO: 13581 - RNA, 20 nt, synthetic construct
  source 1..20: mol_type = other RNA
gcactcttcactttggggaa

SEQ ID NO: 13582 - RNA, 20 nt, synthetic construct
  source 1..20: mol_type = other RNA
gcagggcactcttcactttg

SEQ ID NO: 13583 - RNA, 20 nt, synthetic construct
  source 1..20: mol_type = other RNA
ggcagggcactcttcacttt

SEQ ID NO: 13584 - RNA, 20 nt, synthetic construct
  source 1..20: mol_type = other RNA
gggcagggcactcttcactt

SEQ ID NO: 13585 - RNA, 20 nt, synthetic construct
  source 1..20: mol_type = other RNA
gaagagtgccctgccctcac

SEQ ID NO: 13586 - RNA, 20 nt, synthetic construct
  source 1..20: mol_type = other RNA
aagagtgccctgccctcact

SEQ ID NO: 13587 - RNA, 20 nt, synthetic construct
  source 1..20: mol_type = other RNA
ggcagagcccagtgagggca

SEQ ID NO: 13588 - RNA, 20 nt, synthetic construct
  source 1..20: mol_type = other RNA
gggcagagcccagtgagggc

SEQ ID NO: 13589 - RNA, 20 nt, synthetic construct
  source 1..20: mol_type = other RNA
gaatgggcagagcccagtga

SEQ ID NO: 13590 - RNA, 20 nt, synthetic construct
  source 1..20: mol_type = other RNA
ggaatgggcagagcccagtg

SEQ ID NO: 13591 - RNA, 20 nt, synthetic construct
  source 1..20: mol_type = other RNA
gctctgcccattcctcaccg

SEQ ID NO: 13592 - RNA, 20 nt, synthetic construct
  source 1..20: mol_type = other RNA
agtataccacggtgaggaat

SEQ ID NO: 13593 - RNA, 20 nt, synthetic construct
  source 1..20: mol_type = other RNA
aagtataccacggtgaggaa

SEQ ID NO: 13594 - RNA, 20 nt, synthetic construct
  source 1..20: mol_type = other RNA
ccgtggtatacttgcccagc

SEQ ID NO: 13595 - RNA, 20 nt, synthetic construct
  source 1..20: mol_type = other RNA
ccagctgggcaagtatacca

SEQ ID NO: 13596 - RNA, 20 nt, synthetic construct
  source 1..20: mol_type = other RNA
cttgcccagctggcagagcg

SEQ ID NO: 13597 - RNA, 20 nt, synthetic construct
  source 1..20: mol_type = other RNA
ttgcccagctggcagagcga

SEQ ID NO: 13598 - RNA, 20 nt, synthetic construct
  source 1..20: mol_type = other RNA
tgcccagctggcagagcgag

SEQ ID NO: 13599 - RNA, 20 nt, synthetic construct
  source 1..20: mol_type = other RNA
ttcccctcgctctgccagct

SEQ ID NO: 13600 - RNA, 20 nt, synthetic construct
  source 1..20: mol_type = other RNA
tttcccctcgctctgccagc

SEQ ID NO: 13601 - RNA, 20 nt, synthetic construct
  source 1..20: mol_type = other RNA
gcgaggggaaagtctcctga

SEQ ID NO: 13602 - RNA, 20 nt, synthetic construct
  source 1..20: mol_type = other RNA
cgaggggaaagtctcctgat

SEQ ID NO: 13603 - RNA, 20 nt, synthetic construct
  source 1..20: mol_type = other RNA
ctgatgggctttgctgacct

SEQ ID NO: 13604 - RNA, 20 nt, synthetic construct
  source 1..20: mol_type = other RNA
caaggtcagcaaagcccatc

SEQ ID NO: 13605 - RNA, 20 nt, synthetic construct
  source 1..20: mol_type = other RNA
gtgatgagctcttctaactg

SEQ ID NO: 13606 - RNA, 20 nt, synthetic construct
  source 1..20: mol_type = other RNA
tgatgagctcttctaactga

SEQ ID NO: 13607 - RNA, 20 nt, synthetic construct
  source 1..20: mol_type = other RNA
gggctcagctcatagctgtc

SEQ ID NO: 13608 - RNA, 20 nt, synthetic construct
  source 1..20: mol_type = other RNA
agaaagaggtgaaggaagaa

SEQ ID NO: 13609 - RNA, 20 nt, synthetic construct
  source 1..20: mol_type = other RNA
aagaaagaggtgaaggaaga

SEQ ID NO: 13610 - RNA, 20 nt, synthetic construct
  source 1..20: mol_type = other RNA
caagaagaagaaagaggtga

SEQ ID NO: 13611 - RNA, 20 nt, synthetic construct
  source 1..20: mol_type = other RNA
cctctttcttcttcttgttc

SEQ ID NO: 13612 - RNA, 20 nt, synthetic construct
  source 1..20: mol_type = other RNA
ccggaacaagaagaagaaag

SEQ ID NO: 13613 - RNA, 20 nt, synthetic construct
  source 1..20: mol_type = other RNA
cggtcatttcgcacagcttg

SEQ ID NO: 13614 - RNA, 20 nt, synthetic construct
  source 1..20: mol_type = other RNA
ggtcatttcgcacagcttgt

SEQ ID NO: 13615 - RNA, 20 nt, synthetic construct
  source 1..20: mol_type = other RNA
catttcgcacagcttgtggg

SEQ ID NO: 13616 - RNA, 20 nt, synthetic construct
  source 1..20: mol_type = other RNA
ttcgcacagcttgtgggtgg

SEQ ID NO: 13617 - RNA, 20 nt, synthetic construct
  source 1..20: mol_type = other RNA
agcttgtgggtggaggcgca

SEQ ID NO: 13618 - RNA, 20 nt, synthetic construct
  source 1..20: mol_type = other RNA
gtgggtggaggcgcaaggag

SEQ ID NO: 13619 - RNA, 20 nt, synthetic construct
  source 1..20: mol_type = other RNA
tgggtggaggcgcaaggaga

SEQ ID NO: 13620 - RNA, 20 nt, synthetic construct
  source 1..20: mol_type = other RNA
ggaggcgcaaggagagggtc

SEQ ID NO: 13621 - RNA, 20 nt, synthetic construct
  source 1..20: mol_type = other RNA
ggaccctcagagcctccctt

SEQ ID NO: 13622 - RNA, 20 nt, synthetic construct
  source 1..20: mol_type = other RNA
gaccctcagagcctcccttt

SEQ ID NO: 13623 - RNA, 20 nt, synthetic construct
  source 1..20: mol_type = other RNA
cacccaaagggaggctctga

SEQ ID NO: 13624 - RNA, 20 nt, synthetic construct
  source 1..20: mol_type = other RNA
acacccaaagggaggctctg

SEQ ID NO: 13625 - RNA, 20 nt, synthetic construct
  source 1..20: mol_type = other RNA
gagagaggacacccaaaggg

SEQ ID NO: 13626 - RNA, 20 nt, synthetic construct
  source 1..20: mol_type = other RNA
ggtgagagaggacacccaaa

SEQ ID NO: 13627 - RNA, 20 nt, synthetic construct
  source 1..20: mol_type = other RNA
gggtgagagaggacacccaa

SEQ ID NO: 13628 - RNA, 20 nt, synthetic construct
  source 1..20: mol_type = other RNA
atattaaattagggtgagag

SEQ ID NO: 13629 - RNA, 20 nt, synthetic construct
  source 1..20: mol_type = other RNA
ggactgagcatattaaatta

SEQ ID NO: 13630 - RNA, 20 nt, synthetic construct
  source 1..20: mol_type = other RNA
aggactgagcatattaaatt

SEQ ID NO: 13631 - RNA, 20 nt, synthetic construct
  source 1..20: mol_type = other RNA
tatcatgaatatctattctc

SEQ ID NO: 13632 - RNA, 20 nt, synthetic construct
  source 1..20: mol_type = other RNA
gagaatagatattcatgata

SEQ ID NO: 13633 - RNA, 20 nt, synthetic construct
  source 1..20: mol_type = other RNA
cagggcaggccaagtctcag

SEQ ID NO: 13634 - RNA, 20 nt, synthetic construct
  source 1..20: mol_type = other RNA
ctgagacttggcctgccctg

SEQ ID NO: 13635 - RNA, 20 nt, synthetic construct
  source 1..20: mol_type = other RNA
tctgagacttggcctgccct

SEQ ID NO: 13636 - RNA, 20 nt, synthetic construct
  source 1..20: mol_type = other RNA
ctctgagacttggcctgccc

SEQ ID NO: 13637 - RNA, 20 nt, synthetic construct
  source 1..20: mol_type = other RNA
caggccaagtctcagaggtc

SEQ ID NO: 13638 - RNA, 20 nt, synthetic construct
  source 1..20: mol_type = other RNA
aggccaagtctcagaggtca

SEQ ID NO: 13639 - RNA, 20 nt, synthetic construct
  source 1..20: mol_type = other RNA
agtctcagaggtcagggaag

SEQ ID NO: 13640 - RNA, 20 nt, synthetic construct
  source 1..20: mol_type = other RNA
gtctcagaggtcagggaagt

SEQ ID NO: 13641 - RNA, 20 nt, synthetic construct
  source 1..20: mol_type = other RNA
cttccctgacctctgagact

SEQ ID NO: 13642 - RNA, 20 nt, synthetic construct
  source 1..20: mol_type = other RNA
agaggtcagggaagtgggag

SEQ ID NO: 13643 - RNA, 20 nt, synthetic construct
  source 1..20: mol_type = other RNA
agggaagtgggagtggccag

SEQ ID NO: 13644 - RNA, 20 nt, synthetic construct
  source 1..20: mol_type = other RNA
tgggagtggccagaggaaag

SEQ ID NO: 13645 - RNA, 20 nt, synthetic construct
  source 1..20: mol_type = other RNA
gggagtggccagaggaaaga

SEQ ID NO: 13646 - RNA, 20 nt, synthetic construct
  source 1..20: mol_type = other RNA
ggctgtggccctctttcctc

SEQ ID NO: 13647 - RNA, 20 nt, synthetic construct
  source 1..20: mol_type = other RNA
gaaagagggccacagccata

SEQ ID NO: 13648 - RNA, 20 nt, synthetic construct
  source 1..20: mol_type = other RNA
gagggccacagccatagggt

SEQ ID NO: 13649 - RNA, 20 nt, synthetic construct
  source 1..20: mol_type = other RNA
tcggtcctaccctatggctg

SEQ ID NO: 13650 - RNA, 20 nt, synthetic construct
  source 1..20: mol_type = other RNA
agcacttcggtcctacccta

SEQ ID NO: 13651 - RNA, 20 nt, synthetic construct
  source 1..20: mol_type = other RNA
aagtgctcctgcccaagcca

SEQ ID NO: 13652 - RNA, 20 nt, synthetic construct
  source 1..20: mol_type = other RNA
tggcttgggcaggagcactt

SEQ ID NO: 13653 - RNA, 20 nt, synthetic construct
  source 1..20: mol_type = other RNA
gctcctgcccaagccaagga

SEQ ID NO: 13654 - RNA, 20 nt, synthetic construct
  source 1..20: mol_type = other RNA
ctgccatccttggcttgggc

SEQ ID NO: 13655 - RNA, 20 nt, synthetic construct
  source 1..20: mol_type = other RNA
taggctgccatccttggctt

SEQ ID NO: 13656 - RNA, 20 nt, synthetic construct
  source 1..20: mol_type = other RNA
gtaggctgccatccttggct

SEQ ID NO: 13657 - RNA, 20 nt, synthetic construct
  source 1..20: mol_type = other RNA
ggatggcagcctaccttcct

SEQ ID NO: 13658 - RNA, 20 nt, synthetic construct
  source 1..20: mol_type = other RNA
ggaaggtaggctgccatcct

SEQ ID NO: 13659 - RNA, 20 nt, synthetic construct
  source 1..20: mol_type = other RNA
tgggcatgtccaaggaaggt

SEQ ID NO: 13660 - RNA, 20 nt, synthetic construct
  source 1..20: mol_type = other RNA
gaagtgggcatgtccaagga

SEQ ID NO: 13661 - RNA, 20 nt, synthetic construct
  source 1..20: mol_type = other RNA
cttcgaagtgggcatgtcca

SEQ ID NO: 13662 - RNA, 20 nt, synthetic construct
  source 1..20: mol_type = other RNA
cttcgaagcacttctgtagc

SEQ ID NO: 13663 - RNA, 20 nt, synthetic construct
  source 1..20: mol_type = other RNA
ctacagaagtgcttcgaagt

SEQ ID NO: 13664 - RNA, 20 nt, synthetic construct
  source 1..20: mol_type = other RNA
gctacagaagtgcttcgaag

SEQ ID NO: 13665 - RNA, 20 nt, synthetic construct
  source 1..20: mol_type = other RNA
acttctgtagccggcagtac

SEQ ID NO: 13666 - RNA, 20 nt, synthetic construct
  source 1..20: mol_type = other RNA
gcagtactggcagcgattcc

SEQ ID NO: 13667 - RNA, 20 nt, synthetic construct
  source 1..20: mol_type = other RNA
ggaatcgctgccagtactgc

SEQ ID NO: 13668 - RNA, 20 nt, synthetic construct
  source 1..20: mol_type = other RNA
gtatcatcaacaaggtgacc

SEQ ID NO: 13669 - RNA, 20 nt, synthetic construct
  source 1..20: mol_type = other RNA
caaaaactgtatcatcaaca

SEQ ID NO: 13670 - RNA, 20 nt, synthetic construct
  source 1..20: mol_type = other RNA
tgatgatacagtttttgtcg

SEQ ID NO: 13671 - RNA, 20 nt, synthetic construct
  source 1..20: mol_type = other RNA
acgtgtacaccatgttcttc

SEQ ID NO: 13672 - RNA, 20 nt, synthetic construct
  source 1..20: mol_type = other RNA
ccatgttcttctggatgctt

SEQ ID NO: 13673 - RNA, 20 nt, synthetic construct
  source 1..20: mol_type = other RNA
ccgaagcatccagaagaaca

SEQ ID NO: 13674 - RNA, 20 nt, synthetic construct
  source 1..20: mol_type = other RNA
tgcttcggcgaaagaagccc

SEQ ID NO: 13675 - RNA, 20 nt, synthetic construct
  source 1..20: mol_type = other RNA
cgaaagaagccctggagttg

SEQ ID NO: 13676 - RNA, 20 nt, synthetic construct
  source 1..20: mol_type = other RNA
gaaagaagccctggagttga

SEQ ID NO: 13677 - RNA, 20 nt, synthetic construct
  source 1..20: mol_type = other RNA
tggagttgagggaaagagag

SEQ ID NO: 13678 - RNA, 20 nt, synthetic construct
  source 1..20: mol_type = other RNA
ggagttgagggaaagagaga

SEQ ID NO: 13679 - RNA, 20 nt, synthetic construct
  source 1..20: mol_type = other RNA
ctctctttccctcaactcca

SEQ ID NO: 13680 - RNA, 20 nt, synthetic construct
  source 1..20: mol_type = other RNA
tctctctttccctcaactcc

SEQ ID NO: 13681 - RNA, 20 nt, synthetic construct
  source 1..20: mol_type = other RNA
gggcctctgaagcacaatgc

SEQ ID NO: 13682 - RNA, 20 nt, synthetic construct
  source 1..20: mol_type = other RNA
ggcctctgaagcacaatgct

SEQ ID NO: 13683 - RNA, 20 nt, synthetic construct
  source 1..20: mol_type = other RNA
ctcccagcattgtgcttcag

SEQ ID NO: 13684 - RNA, 20 nt, synthetic construct
  source 1..20: mol_type = other RNA
tgggagtaccagcctctcac

SEQ ID NO: 13685 - RNA, 20 nt, synthetic construct
  source 1..20: mol_type = other RNA
cagcctctcactggccttgc

SEQ ID NO: 13686 - RNA, 20 nt, synthetic construct
  source 1..20: mol_type = other RNA
ctgcaaggccagtgagaggc

SEQ ID NO: 13687 - RNA, 20 nt, synthetic construct
  source 1..20: mol_type = other RNA
caacctgcaaggccagtgag

SEQ ID NO: 13688 - RNA, 20 nt, synthetic construct
  source 1..20: mol_type = other RNA
caggcttggggcaacctgca

SEQ ID NO: 13689 - RNA, 20 nt, synthetic construct
  source 1..20: mol_type = other RNA
aatagattaggtcaggcttg

SEQ ID NO: 13690 - RNA, 20 nt, synthetic construct
  source 1..20: mol_type = other RNA
taatagattaggtcaggctt

SEQ ID NO: 13691 - RNA, 20 nt, synthetic construct
  source 1..20: mol_type = other RNA
ttaatagattaggtcaggct

SEQ ID NO: 13692 - RNA, 20 nt, synthetic construct
  source 1..20: mol_type = other RNA
ggtggttaatagattaggtc

SEQ ID NO: 13693 - RNA, 20 nt, synthetic construct
  source 1..20: mol_type = other RNA
acataggtggttaatagatt

SEQ ID NO: 13694 - RNA, 20 nt, synthetic construct
  source 1..20: mol_type = other RNA
agcactgctttgcacatagg

SEQ ID NO: 13695 - RNA, 20 nt, synthetic construct
  source 1..20: mol_type = other RNA
agcagcactgctttgcacat

SEQ ID NO: 13696 - RNA, 20 nt, synthetic construct
  source 1..20: mol_type = other RNA
agacacagcatctgtgtgcc

SEQ ID NO: 13697 - RNA, 20 nt, synthetic construct
  source 1..20: mol_type = other RNA
gcctggtctctcatcttact

SEQ ID NO: 13698 - RNA, 20 nt, synthetic construct
  source 1..20: mol_type = other RNA
cctggtctctcatcttacta

SEQ ID NO: 13699 - RNA, 20 nt, synthetic construct
  source 1..20: mol_type = other RNA
ccctagtaagatgagagacc

SEQ ID NO: 13700 - RNA, 20 nt, synthetic construct
  source 1..20: mol_type = other RNA
tctcatcttactagggtaac

SEQ ID NO: 13701 - RNA, 20 nt, synthetic construct
  source 1..20: mol_type = other RNA
tggtgggagtgggcagacgg

SEQ ID NO: 13702 - RNA, 20 nt, synthetic construct
  source 1..20: mol_type = other RNA
gtggtgggagtgggcagacg

SEQ ID NO: 13703 - RNA, 20 nt, synthetic construct
  source 1..20: mol_type = other RNA
cgtggtgggagtgggcagac

SEQ ID NO: 13704 - RNA, 20 nt, synthetic construct
  source 1..20: mol_type = other RNA
acgtggtgggagtgggcaga

SEQ ID NO: 13705 - RNA, 20 nt, synthetic construct
  source 1..20: mol_type = other RNA
ggtgtgtacgtggtgggagt

SEQ ID NO: 13706 - RNA, 20 nt, synthetic construct
  source 1..20: mol_type = other RNA
aggtgtgtacgtggtgggag

SEQ ID NO: 13707 - RNA, 20 nt, synthetic construct
  source 1..20: mol_type = other RNA
ctgcaaggtgtgtacgtggt

SEQ ID NO: 13708 - RNA, 20 nt, synthetic construct
  source 1..20: mol_type = other RNA
gctgcaaggtgtgtacgtgg

SEQ ID NO: 13709 - RNA, 20 nt, synthetic construct
  source 1..20: mol_type = other RNA
aaggctgcaaggtgtgtacg

SEQ ID NO: 13710 - RNA, 20 nt, synthetic construct
  source 1..20: mol_type = other RNA
cagctcttgtgaaggctgca

SEQ ID NO: 13711 - RNA, 20 nt, synthetic construct
  source 1..20: mol_type = other RNA
cacaagagctgaccccatag

SEQ ID NO: 13712 - RNA, 20 nt, synthetic construct
  source 1..20: mol_type = other RNA
tatggggtcagctcttgtga

SEQ ID NO: 13713 - RNA, 20 nt, synthetic construct
  source 1..20: mol_type = other RNA
gaccccatagtggtagccag

SEQ ID NO: 13714 - RNA, 20 nt, synthetic construct
  source 1..20: mol_type = other RNA
gtcctctggctaccactatg

SEQ ID NO: 13715 - RNA, 20 nt, synthetic construct
  source 1..20: mol_type = other RNA
agtcctctggctaccactat

SEQ ID NO: 13716 - RNA, 20 nt, synthetic construct
  source 1..20: mol_type = other RNA
aagtcctctggctaccacta

SEQ ID NO: 13717 - RNA, 20 nt, synthetic construct
  source 1..20: mol_type = other RNA
gtgtgcaatgacaagtcctc

SEQ ID NO: 13718 - RNA, 20 nt, synthetic construct
  source 1..20: mol_type = other RNA
ttgtcattgcacacgaagca

SEQ ID NO: 13719 - RNA, 20 nt, synthetic construct
  source 1..20: mol_type = other RNA
aagcatggcttgtagacccg

SEQ ID NO: 13720 - RNA, 20 nt, synthetic construct
  source 1..20: mol_type = other RNA
catggcttgtagacccgagg

SEQ ID NO: 13721 - RNA, 20 nt, synthetic construct
  source 1..20: mol_type = other RNA
ggcttgtagacccgaggagg

SEQ ID NO: 13722 - RNA, 20 nt, synthetic construct
  source 1..20: mol_type = other RNA
ttgtagacccgaggaggcgg

SEQ ID NO: 13723 - RNA, 20 nt, synthetic construct
  source 1..20: mol_type = other RNA
tgtagacccgaggaggcgga

SEQ ID NO: 13724 - RNA, 20 nt, synthetic construct
  source 1..20: mol_type = other RNA
gtagacccgaggaggcggag

SEQ ID NO: 13725 - RNA, 20 nt, synthetic construct
  source 1..20: mol_type = other RNA
tagacccgaggaggcggagg

SEQ ID NO: 13726 - RNA, 20 nt, synthetic construct
  source 1..20: mol_type = other RNA
ccgaggaggcggagggggcg

SEQ ID NO: 13727 - RNA, 20 nt, synthetic construct
  source 1..20: mol_type = other RNA
cgaggaggcggagggggcga

SEQ ID NO: 13728 - RNA, 20 nt, synthetic construct
  source 1..20: mol_type = other RNA
ctcgccccctccgcctcctc

SEQ ID NO: 13729 - RNA, 20 nt, synthetic construct
  source 1..20: mol_type = other RNA
cctcgccccctccgcctcct

SEQ ID NO: 13730 - RNA, 20 nt, synthetic construct
  source 1..20: mol_type = other RNA
cggagggggcgagggcgagc

SEQ ID NO: 13731 - RNA, 20 nt, synthetic construct
  source 1..20: mol_type = other RNA
ggagggggcgagggcgagct

SEQ ID NO: 13732 - RNA, 20 nt, synthetic construct
  source 1..20: mol_type = other RNA
gggcaccatctcctctgagc

SEQ ID NO: 13733 - RNA, 20 nt, synthetic construct
  source 1..20: mol_type = other RNA
gagcaccagctcagaggaga

SEQ ID NO: 13734 - RNA, 20 nt, synthetic construct
  source 1..20: mol_type = other RNA
gacacagagcaccagctcag

SEQ ID NO: 13735 - RNA, 20 nt, synthetic construct
  source 1..20: mol_type = other RNA
gtgctctgtgtctccaccgc

SEQ ID NO: 13736 - RNA, 20 nt, synthetic construct
  source 1..20: mol_type = other RNA
tgctctgtgtctccaccgct

SEQ ID NO: 13737 - RNA, 20 nt, synthetic construct
  source 1..20: mol_type = other RNA
tctgtgtctccaccgctggg

SEQ ID NO: 13738 - RNA, 20 nt, synthetic construct
  source 1..20: mol_type = other RNA
ctgtgtctccaccgctggga

SEQ ID NO: 13739 - RNA, 20 nt, synthetic construct
  source 1..20: mol_type = other RNA
cactgcttccctcccagcgg

SEQ ID NO: 13740 - RNA, 20 nt, synthetic construct
  source 1..20: mol_type = other RNA
catcactgcttccctcccag

SEQ ID NO: 13741 - RNA, 20 nt, synthetic construct
  source 1..20: mol_type = other RNA
ggagggaagcagtgatgtga

SEQ ID NO: 13742 - RNA, 20 nt, synthetic construct
  source 1..20: mol_type = other RNA
gaagcagtgatgtgagggtc

SEQ ID NO: 13743 - RNA, 20 nt, synthetic construct
  source 1..20: mol_type = other RNA
aagcagtgatgtgagggtca

SEQ ID NO: 13744 - RNA, 20 nt, synthetic construct
  source 1..20: mol_type = other RNA
agcagtgatgtgagggtcag

SEQ ID NO: 13745 - RNA, 20 nt, synthetic construct
  source 1..20: mol_type = other RNA
gatgtgagggtcaggggaga

SEQ ID NO: 13746 - RNA, 20 nt, synthetic construct
  source 1..20: mol_type = other RNA
gaaggaccccacagacctcc

SEQ ID NO: 13747 - RNA, 20 nt, synthetic construct
  source 1..20: mol_type = other RNA
aggaagcctggaggtctgtg

SEQ ID NO: 13748 - RNA, 20 nt, synthetic construct
  source 1..20: mol_type = other RNA
gaggaagcctggaggtctgt

SEQ ID NO: 13749 - RNA, 20 nt, synthetic construct
  source 1..20: mol_type = other RNA
tgaggaagcctggaggtctg

SEQ ID NO: 13750 - RNA, 20 nt, synthetic construct
  source 1..20: mol_type = other RNA
tgtgtgatgaggaagcctgg

SEQ ID NO: 13751 - RNA, 20 nt, synthetic construct
  source 1..20: mol_type = other RNA
gtgtgtgtgatgaggaagcc

SEQ ID NO: 13752 - RNA, 20 nt, synthetic construct
  source 1..20: mol_type = other RNA
cacatggggtgtgtgtgatg

SEQ ID NO: 13753 - RNA, 20 nt, synthetic construct
  source 1..20: mol_type = other RNA
ccccatgtgcatttgttcct

SEQ ID NO: 13754 - RNA, 20 nt, synthetic construct
  source 1..20: mol_type = other RNA
ccaaggaacaaatgcacatg

SEQ ID NO: 13755 - RNA, 20 nt, synthetic construct
  source 1..20: mol_type = other RNA
gccaaggaacaaatgcacat

SEQ ID NO: 13756 - RNA, 20 nt, synthetic construct
  source 1..20: mol_type = other RNA
ggccaaggaacaaatgcaca

SEQ ID NO: 13757 - RNA, 20 nt, synthetic construct
  source 1..20: mol_type = other RNA
gcatttgttccttggcccac

SEQ ID NO: 13758 - RNA, 20 nt, synthetic construct
  source 1..20: mol_type = other RNA
tggctgtcaccagtgggcca

SEQ ID NO: 13759 - RNA, 20 nt, synthetic construct
  source 1..20: mol_type = other RNA
tagtgatggctgtcaccagt

SEQ ID NO: 13760 - RNA, 20 nt, synthetic construct
  source 1..20: mol_type = other RNA
gtagtgatggctgtcaccag

SEQ ID NO: 13761 - RNA, 20 nt, synthetic construct
  source 1..20: mol_type = other RNA
gccctttctatgtaaggtac

SEQ ID NO: 13762 - RNA, 20 nt, synthetic construct
  source 1..20: mol_type = other RNA
cttctggccctttctatgta

SEQ ID NO: 13763 - RNA, 20 nt, synthetic construct
  source 1..20: mol_type = other RNA
gaggtgcaaggaggagcttc

SEQ ID NO: 13764 - RNA, 20 nt, synthetic construct
  source 1..20: mol_type = other RNA
agtggaactgaggtgcaagg

SEQ ID NO: 13765 - RNA, 20 nt, synthetic construct
  source 1..20: mol_type = other RNA
aagagtggaactgaggtgca

SEQ ID NO: 13766 - RNA, 20 nt, synthetic construct
  source 1..20: mol_type = other RNA
tcagttccactctttacaca

SEQ ID NO: 13767 - RNA, 20 nt, synthetic construct
  source 1..20: mol_type = other RNA
gtgtgtaaagagtggaactg

SEQ ID NO: 13768 - RNA, 20 nt, synthetic construct
  source 1..20: mol_type = other RNA
ctctttccgtgtgtaaagag

SEQ ID NO: 13769 - RNA, 20 nt, synthetic construct
  source 1..20: mol_type = other RNA
tgtagggtgcaggagagggt

SEQ ID NO: 13770 - RNA, 20 nt, synthetic construct
  source 1..20: mol_type = other RNA
gtgtagggtgcaggagaggg

SEQ ID NO: 13771 - RNA, 20 nt, synthetic construct
  source 1..20: mol_type = other RNA
ggggtgtagggtgcaggaga

SEQ ID NO: 13772 - RNA, 20 nt, synthetic construct
  source 1..20: mol_type = other RNA
tggggtgtagggtgcaggag

SEQ ID NO: 13773 - RNA, 20 nt, synthetic construct
  source 1..20: mol_type = other RNA
tgcaccctacaccccagccc

SEQ ID NO: 13774 - RNA, 20 nt, synthetic construct
  source 1..20: mol_type = other RNA
ggggctggggtgtagggtgc

SEQ ID NO: 13775 - RNA, 20 nt, synthetic construct
  source 1..20: mol_type = other RNA
tacaccccagccccggactc

SEQ ID NO: 13776 - RNA, 20 nt, synthetic construct
  source 1..20: mol_type = other RNA
gagtccggggctggggtgta

SEQ ID NO: 13777 - RNA, 20 nt, synthetic construct
  source 1..20: mol_type = other RNA
ggagtccggggctggggtgt

SEQ ID NO: 13778 - RNA, 20 nt, synthetic construct
  source 1..20: mol_type = other RNA
ggtaccggagtccggggctg

SEQ ID NO: 13779 - RNA, 20 nt, synthetic construct
  source 1..20: mol_type = other RNA
aggtaccggagtccggggct

SEQ ID NO: 13780 - RNA, 20 nt, synthetic construct
  source 1..20: mol_type = other RNA
taggtaccggagtccggggc

SEQ ID NO: 13781 - RNA, 20 nt, synthetic construct
  source 1..20: mol_type = other RNA
aatgtaggtaccggagtccg

SEQ ID NO: 13782 - RNA, 20 nt, synthetic construct
  source 1..20: mol_type = other RNA
caatgtaggtaccggagtcc

SEQ ID NO: 13783 - RNA, 20 nt, synthetic construct
  source 1..20: mol_type = other RNA
gcaatgtaggtaccggagtc

SEQ ID NO: 13784 - RNA, 20 nt, synthetic construct
  source 1..20: mol_type = other RNA
ccggtacctacattgcaggc

SEQ ID NO: 13785 - RNA, 20 nt, synthetic construct
  source 1..20: mol_type = other RNA
gtacctacattgcaggctgg

SEQ ID NO: 13786 - RNA, 20 nt, synthetic construct
  source 1..20: mol_type = other RNA
tacctacattgcaggctggc

SEQ ID NO: 13787 - RNA, 20 nt, synthetic construct
  source 1..20: mol_type = other RNA
ccagcctgcaatgtaggtac

SEQ ID NO: 13788 - RNA, 20 nt, synthetic construct
  source 1..20: mol_type = other RNA
cattgcaggctggcgggttg

SEQ ID NO: 13789 - RNA, 20 nt, synthetic construct
  source 1..20: mol_type = other RNA
aacccgccagcctgcaatgt

SEQ ID NO: 13790 - RNA, 20 nt, synthetic construct
  source 1..20: mol_type = other RNA
caggctggcgggttgcggcc

SEQ ID NO: 13791 - RNA, 20 nt, synthetic construct
  source 1..20: mol_type = other RNA
ccaggcaaaagattcaagtc

SEQ ID NO: 13792 - RNA, 20 nt, synthetic construct
  source 1..20: mol_type = other RNA
ccggacttgaatcttttgcc

SEQ ID NO: 13793 - RNA, 20 nt, synthetic construct
  source 1..20: mol_type = other RNA
agattcaagtccggcgaaac

SEQ ID NO: 13794 - RNA, 20 nt, synthetic construct
  source 1..20: mol_type = other RNA
tccggcgaaacaggagccgc

SEQ ID NO: 13795 - RNA, 20 nt, synthetic construct
  source 1..20: mol_type = other RNA
ggcgaaacaggagccgccgg

SEQ ID NO: 13796 - RNA, 20 nt, synthetic construct
  source 1..20: mol_type = other RNA
accggcggctcctgtttcgc

SEQ ID NO: 13797 - RNA, 20 nt, synthetic construct
  source 1..20: mol_type = other RNA
ttgctgcgcagagccaccgg

SEQ ID NO: 13798 - RNA, 20 nt, synthetic construct
  source 1..20: mol_type = other RNA
ggcttgctgcgcagagccac

SEQ ID NO: 13799 - RNA, 20 nt, synthetic construct
  source 1..20: mol_type = other RNA
tctgcgcagcaagccggccc

SEQ ID NO: 13800 - RNA, 20 nt, synthetic construct
  source 1..20: mol_type = other RNA
ctgcgcagcaagccggcccc

SEQ ID NO: 13801 - RNA, 20 nt, synthetic construct
  source 1..20: mol_type = other RNA
cagcaagccggccccgggcc

SEQ ID NO: 13802 - RNA, 20 nt, synthetic construct
  source 1..20: mol_type = other RNA
ggggcggccgggcccggggc

SEQ ID NO: 13803 - RNA, 20 nt, synthetic construct
  source 1..20: mol_type = other RNA
gtacggggcggccgggcccg

SEQ ID NO: 13804 - RNA, 20 nt, synthetic construct
  source 1..20: mol_type = other RNA
tgtacggggcggccgggccc

SEQ ID NO: 13805 - RNA, 20 nt, synthetic construct
  source 1..20: mol_type = other RNA
ctgtacggggcggccgggcc

SEQ ID NO: 13806 - RNA, 20 nt, synthetic construct
  source 1..20: mol_type = other RNA
gccgccccgtacagccgtcg

SEQ ID NO: 13807 - RNA, 20 nt, synthetic construct
  source 1..20: mol_type = other RNA
gacggctgtacggggcggcc

SEQ ID NO: 13808 - RNA, 20 nt, synthetic construct
  source 1..20: mol_type = other RNA
cgacggctgtacggggcggc

SEQ ID NO: 13809 - RNA, 20 nt, synthetic construct
  source 1..20: mol_type = other RNA
ccgtacagccgtcgcggacc

SEQ ID NO: 13810 - RNA, 20 nt, synthetic construct
  source 1..20: mol_type = other RNA
cgtacagccgtcgcggaccc

SEQ ID NO: 13811 - RNA, 20 nt, synthetic construct
  source 1..20: mol_type = other RNA
gtacagccgtcgcggacccg

SEQ ID NO: 13812 - RNA, 20 nt, synthetic construct
  source 1..20: mol_type = other RNA
gggtccgcgacggctgtacg

SEQ ID NO: 13813 - RNA, 20 nt, synthetic construct
  source 1..20: mol_type = other RNA
cgggtccgcgacggctgtac

SEQ ID NO: 13814 - RNA, 20 nt, synthetic construct
  source 1..20: mol_type = other RNA
ccgggtccgcgacggctgta

SEQ ID NO: 13815 - RNA, 20 nt, synthetic construct
  source 1..20: mol_type = other RNA
cgtttgccccgggtccgcga

SEQ ID NO: 13816 - RNA, 20 nt, synthetic construct
  source 1..20: mol_type = other RNA
tgtatggaaacgtttgcccc

SEQ ID NO: 13817 - RNA, 20 nt, synthetic construct
  source 1..20: mol_type = other RNA
ctgtatggaaacgtttgccc

SEQ ID NO: 13818 - RNA, 20 nt, synthetic construct
  source 1..20: mol_type = other RNA
tacagtcgtacatcgcgacc

SEQ ID NO: 13819 - RNA, 20 nt, synthetic construct
  source 1..20: mol_type = other RNA
ggtcgcgatgtacgactgta

SEQ ID NO: 13820 - RNA, 20 nt, synthetic construct
  source 1..20: mol_type = other RNA
tacatcgcgacccggcttga

SEQ ID NO: 13821 - RNA, 20 nt, synthetic construct
  source 1..20: mol_type = other RNA
acatcgcgacccggcttgaa

SEQ ID NO: 13822 - RNA, 20 nt, synthetic construct
  source 1..20: mol_type = other RNA
gacccggcttgaagggaaac

SEQ ID NO: 13823 - RNA, 20 nt, synthetic construct
  source 1..20: mol_type = other RNA
acccggcttgaagggaaact

SEQ ID NO: 13824 - RNA, 20 nt, synthetic construct
  source 1..20: mol_type = other RNA
acccagtttcccttcaagcc

SEQ ID NO: 13825 - RNA, 20 nt, synthetic construct
  source 1..20: mol_type = other RNA
cacccagtttcccttcaagc

SEQ ID NO: 13826 - RNA, 20 nt, synthetic construct
  source 1..20: mol_type = other RNA
actgggtgctggaaacacca

SEQ ID NO: 13827 - RNA, 20 nt, synthetic construct
  source 1..20: mol_type = other RNA
gggaatcggctgcgggtcct

SEQ ID NO: 13828 - RNA, 20 nt, synthetic construct
  source 1..20: mol_type = other RNA
gaggagggggaatcggctgc

SEQ ID NO: 13829 - RNA, 20 nt, synthetic construct
  source 1..20: mol_type = other RNA
gccgattccccctcctcccc

SEQ ID NO: 13830 - RNA, 20 nt, synthetic construct
  source 1..20: mol_type = other RNA
gattccccctcctcccccgg

SEQ ID NO: 13831 - RNA, 20 nt, synthetic construct
  source 1..20: mol_type = other RNA
gccgggggaggagggggaat

SEQ ID NO: 13832 - RNA, 20 nt, synthetic construct
  source 1..20: mol_type = other RNA
ggcgccgccgggggaggagg

SEQ ID NO: 13833 - RNA, 20 nt, synthetic construct
  source 1..20: mol_type = other RNA
gggcgccgccgggggaggag

SEQ ID NO: 13834 - RNA, 20 nt, synthetic construct
  source 1..20: mol_type = other RNA
ggggcgccgccgggggagga

SEQ ID NO: 13835 - RNA, 20 nt, synthetic construct
  source 1..20: mol_type = other RNA
cggggcgccgccgggggagg

SEQ ID NO: 13836 - RNA, 20 nt, synthetic construct
  source 1..20: mol_type = other RNA
gagcggggcgccgccggggg

SEQ ID NO: 13837 - RNA, 20 nt, synthetic construct
  source 1..20: mol_type = other RNA
cggcggcgccccgctccagc

SEQ ID NO: 13838 - RNA, 20 nt, synthetic construct
  source 1..20: mol_type = other RNA
ctggagcggggcgccgccgg

SEQ ID NO: 13839 - RNA, 20 nt, synthetic construct
  source 1..20: mol_type = other RNA
gctggagcggggcgccgccg

SEQ ID NO: 13840 - RNA, 20 nt, synthetic construct
  source 1..20: mol_type = other RNA
cggcgccccgctccagcagg

SEQ ID NO: 13841 - RNA, 20 nt, synthetic construct
  source 1..20: mol_type = other RNA
ctgctggagcggggcgccgc

SEQ ID NO: 13842 - RNA, 20 nt, synthetic construct
  source 1..20: mol_type = other RNA
gcgccccgctccagcagggg

SEQ ID NO: 13843 - RNA, 20 nt, synthetic construct
  source 1..20: mol_type = other RNA
ccccgctccagcaggggggg

SEQ ID NO: 13844 - RNA, 20 nt, synthetic construct
  source 1..20: mol_type = other RNA
cccgctccagcaggggggga

SEQ ID NO: 13845 - RNA, 20 nt, synthetic construct
  source 1..20: mol_type = other RNA
ccgctccagcagggggggag

SEQ ID NO: 13846 - RNA, 20 nt, synthetic construct
  source 1..20: mol_type = other RNA
cgctccagcagggggggagg

SEQ ID NO: 13847 - RNA, 20 nt, synthetic construct
  source 1..20: mol_type = other RNA
cctccccccctgctggagcg

SEQ ID NO: 13848 - RNA, 20 nt, synthetic construct
  source 1..20: mol_type = other RNA
ccctccccccctgctggagc

SEQ ID NO: 13849 - RNA, 20 nt, synthetic construct
  source 1..20: mol_type = other RNA
cccctccccccctgctggag

SEQ ID NO: 13850 - RNA, 20 nt, synthetic construct
  source 1..20: mol_type = other RNA
ccctccccctccccccctgc

SEQ ID NO: 13851 - RNA, 20 nt, synthetic construct
  source 1..20: mol_type = other RNA
gggagggggagggctagcat

SEQ ID NO: 13852 - RNA, 20 nt, synthetic construct
  source 1..20: mol_type = other RNA
ggagggggagggctagcata

SEQ ID NO: 13853 - RNA, 20 nt, synthetic construct
  source 1..20: mol_type = other RNA
ggagggctagcatagggcgc

SEQ ID NO: 13854 - RNA, 20 nt, synthetic construct
  source 1..20: mol_type = other RNA
gagggctagcatagggcgct

SEQ ID NO: 13855 - RNA, 20 nt, synthetic construct
  source 1..20: mol_type = other RNA
atagggcgctgggctgcatg

SEQ ID NO: 13856 - RNA, 20 nt, synthetic construct
  source 1..20: mol_type = other RNA
tagggcgctgggctgcatgc

SEQ ID NO: 13857 - RNA, 20 nt, synthetic construct
  source 1..20: mol_type = other RNA
cgctgggctgcatgcgggta

SEQ ID NO: 13858 - RNA, 20 nt, synthetic construct
  source 1..20: mol_type = other RNA
gctgggctgcatgcgggtaa

SEQ ID NO: 13859 - RNA, 20 nt, synthetic construct
  source 1..20: mol_type = other RNA
ctgggctgcatgcgggtaag

SEQ ID NO: 13860 - RNA, 20 nt, synthetic construct
  source 1..20: mol_type = other RNA
ggctgcatgcgggtaagggg

SEQ ID NO: 13861 - RNA, 20 nt, synthetic construct
  source 1..20: mol_type = other RNA
gctgcatgcgggtaaggggt

SEQ ID NO: 13862 - RNA, 20 nt, synthetic construct
  source 1..20: mol_type = other RNA
gcatgcgggtaaggggtggg

SEQ ID NO: 13863 - RNA, 20 nt, synthetic construct
  source 1..20: mol_type = other RNA
catgcgggtaaggggtgggc

SEQ ID NO: 13864 - RNA, 20 nt, synthetic construct
  source 1..20: mol_type = other RNA
atgcgggtaaggggtgggcg

SEQ ID NO: 13865 - RNA, 20 nt, synthetic construct
  source 1..20: mol_type = other RNA
gtaaggggtgggcggggaag

SEQ ID NO: 13866 - RNA, 20 nt, synthetic construct
  source 1..20: mol_type = other RNA
taaggggtgggcggggaaga

SEQ ID NO: 13867 - RNA, 20 nt, synthetic construct
  source 1..20: mol_type = other RNA
aaggggtgggcggggaagag

SEQ ID NO: 13868 - RNA, 20 nt, synthetic construct
  source 1..20: mol_type = other RNA
aggggtgggcggggaagagg

SEQ ID NO: 13869 - RNA, 20 nt, synthetic construct
  source 1..20: mol_type = other RNA
ggggtgggcggggaagaggg

SEQ ID NO: 13870 - RNA, 20 nt, synthetic construct
  source 1..20: mol_type = other RNA
gaagaggggggatccccagc

SEQ ID NO: 13871 - RNA, 20 nt, synthetic construct
  source 1..20: mol_type = other RNA
aagaggggggatccccagca

SEQ ID NO: 13872 - RNA, 20 nt, synthetic construct
  source 1..20: mol_type = other RNA
agaggggggatccccagcag

SEQ ID NO: 13873 - RNA, 20 nt, synthetic construct
  source 1..20: mol_type = other RNA
ggggatccccagcaggggaa

SEQ ID NO: 13874 - RNA, 20 nt, synthetic construct
  source 1..20: mol_type = other RNA
gggatccccagcaggggaaa

SEQ ID NO: 13875 - RNA, 20 nt, synthetic construct
  source 1..20: mol_type = other RNA
ccccagcaggggaaagggac

SEQ ID NO: 13876 - RNA, 20 nt, synthetic construct
  source 1..20: mol_type = other RNA
cccagcaggggaaagggact

SEQ ID NO: 13877 - RNA, 20 nt, synthetic construct
  source 1..20: mol_type = other RNA
agcaggggaaagggactggg

SEQ ID NO: 13878 - RNA, 20 nt, synthetic construct
  source 1..20: mol_type = other RNA
gcaggggaaagggactgggc

SEQ ID NO: 13879 - RNA, 20 nt, synthetic construct
  source 1..20: mol_type = other RNA
caggggaaagggactgggcg

SEQ ID NO: 13880 - RNA, 20 nt, synthetic construct
  source 1..20: mol_type = other RNA
gcccagtccctttcccctgc

SEQ ID NO: 13881 - RNA, 20 nt, synthetic construct
  source 1..20: mol_type = other RNA
gactgggcggggcgcgaagc

SEQ ID NO: 13882 - RNA, 20 nt, synthetic construct
  source 1..20: mol_type = other RNA
actgggcggggcgcgaagct

SEQ ID NO: 13883 - RNA, 20 nt, synthetic construct
  source 1..20: mol_type = other RNA
ctgggcggggcgcgaagctg

SEQ ID NO: 13884 - RNA, 20 nt, synthetic construct
  source 1..20: mol_type = other RNA
gagctggacggaggctaaag

SEQ ID NO: 13885 - RNA, 20 nt, synthetic construct
  source 1..20: mol_type = other RNA
gcctccgtccagctcttatc

SEQ ID NO: 13886 - RNA, 20 nt, synthetic construct
  source 1..20: mol_type = other RNA
cctccgtccagctcttatct

SEQ ID NO: 13887 - RNA, 20 nt, synthetic construct
  source 1..20: mol_type = other RNA
cccagataagagctggacgg

SEQ ID NO: 13888 - RNA, 20 nt, synthetic construct
  source 1..20: mol_type = other RNA
cagctcttatctgggtgctt

SEQ ID NO: 13889 - RNA, 20 nt, synthetic construct
  source 1..20: mol_type = other RNA
cgaagcacccagataagagc

SEQ ID NO: 13890 - RNA, 20 nt, synthetic construct
  source 1..20: mol_type = other RNA
ggtgcttcggcagctagcac

SEQ ID NO: 13891 - RNA, 20 nt, synthetic construct
  source 1..20: mol_type = other RNA
gtgcttcggcagctagcact

SEQ ID NO: 13892 - RNA, 20 nt, synthetic construct
  source 1..20: mol_type = other RNA
tgcttcggcagctagcactg

SEQ ID NO: 13893 - RNA, 20 nt, synthetic construct
  source 1..20: mol_type = other RNA
ccttttttaaaagcgaagcc

SEQ ID NO: 13894 - RNA, 20 nt, synthetic construct
  source 1..20: mol_type = other RNA
tttttaaaagcgaagcctgg

SEQ ID NO: 13895 - RNA, 20 nt, synthetic construct
  source 1..20: mol_type = other RNA
ttttaaaagcgaagcctgga

SEQ ID NO: 13896 - RNA, 20 nt, synthetic construct
  source 1..20: mol_type = other RNA
ccaggcttcgcttttaaaaa

SEQ ID NO: 13897 - RNA, 20 nt, synthetic construct
  source 1..20: mol_type = other RNA
aaaagcgaagcctggagggg

SEQ ID NO: 13898 - RNA, 20 nt, synthetic construct
  source 1..20: mol_type = other RNA
aaagcgaagcctggaggggt

SEQ ID NO: 13899 - RNA, 20 nt, synthetic construct
  source 1..20: mol_type = other RNA
aagcgaagcctggaggggtg

SEQ ID NO: 13900 - RNA, 20 nt, synthetic construct
  source 1..20: mol_type = other RNA
agcgaagcctggaggggtgg

SEQ ID NO: 13901 - RNA, 20 nt, synthetic construct
  source 1..20: mol_type = other RNA
gcgaagcctggaggggtggg

SEQ ID NO: 13902 - RNA, 20 nt, synthetic construct
  source 1..20: mol_type = other RNA
aagcctggaggggtgggggg

SEQ ID NO: 13903 - RNA, 20 nt, synthetic construct
  source 1..20: mol_type = other RNA
agcctggaggggtggggggt

SEQ ID NO: 13904 - RNA, 20 nt, synthetic construct
  source 1..20: mol_type = other RNA
gcctggaggggtggggggtg

SEQ ID NO: 13905 - RNA, 20 nt, synthetic construct
  source 1..20: mol_type = other RNA
gaggggtggggggtggggct

SEQ ID NO: 13906 - RNA, 20 nt, synthetic construct
  source 1..20: mol_type = other RNA
gccccaccccccacccctcc

SEQ ID NO: 13907 - RNA, 20 nt, synthetic construct
  source 1..20: mol_type = other RNA
gggtggggcttggagagcga

SEQ ID NO: 13908 - RNA, 20 nt, synthetic construct
  source 1..20: mol_type = other RNA
ggtggggcttggagagcgaa

SEQ ID NO: 13909 - RNA, 20 nt, synthetic construct
  source 1..20: mol_type = other RNA
gtggggcttggagagcgaag

SEQ ID NO: 13910 - RNA, 20 nt, synthetic construct
  source 1..20: mol_type = other RNA
tggggcttggagagcgaagg

SEQ ID NO: 13911 - RNA, 20 nt, synthetic construct
  source 1..20: mol_type = other RNA
gcttggagagcgaagggggc

SEQ ID NO: 13912 - RNA, 20 nt, synthetic construct
  source 1..20: mol_type = other RNA
cttggagagcgaagggggcc

SEQ ID NO: 13913 - RNA, 20 nt, synthetic construct
  source 1..20: mol_type = other RNA
gctttgctcatctcggtgcc

SEQ ID NO: 13914 - RNA, 20 nt, synthetic construct
  source 1..20: mol_type = other RNA
gagatgagcaaagctgagag

SEQ ID NO: 13915 - RNA, 20 nt, synthetic construct
  source 1..20: mol_type = other RNA
actctcagctttgctcatct

SEQ ID NO: 13916 - RNA, 20 nt, synthetic construct
  source 1..20: mol_type = other RNA
acatacgtacactcgctccg

SEQ ID NO: 13917 - RNA, 20 nt, synthetic construct
  source 1..20: mol_type = other RNA
ctaagcaagcgcgcgcgccg

SEQ ID NO: 13918 - RNA, 20 nt, synthetic construct
  source 1..20: mol_type = other RNA
gtgcatgcatttatcttatc

SEQ ID NO: 13919 - RNA, 20 nt, synthetic construct
  source 1..20: mol_type = other RNA
tgataagataaatgcatgca

SEQ ID NO: 13920 - RNA, 20 nt, synthetic construct
  source 1..20: mol_type = other RNA
cttgcatatttgcaaattct

SEQ ID NO: 13921 - RNA, 20 nt, synthetic construct
  source 1..20: mol_type = other RNA
gagcacgcatataaaatcat

SEQ ID NO: 13922 - RNA, 20 nt, synthetic construct
  source 1..20: mol_type = other RNA
ttgtgcaaacacaccttgct

SEQ ID NO: 13923 - RNA, 20 nt, synthetic construct
  source 1..20: mol_type = other RNA
tgtgcaaacacaccttgctc

SEQ ID NO: 13924 - RNA, 20 nt, synthetic construct
  source 1..20: mol_type = other RNA
ttgctcgggagaatgcttgc

SEQ ID NO: 13925 - RNA, 20 nt, synthetic construct
  source 1..20: mol_type = other RNA
tgcaagcattctcccgagca

SEQ ID NO: 13926 - RNA, 20 nt, synthetic construct
  source 1..20: mol_type = other RNA
gcatactctccacagctcat

SEQ ID NO: 13927 - RNA, 20 nt, synthetic construct
  source 1..20: mol_type = other RNA
catgcaaagcctatgagctg

SEQ ID NO: 13928 - RNA, 20 nt, synthetic construct
  source 1..20: mol_type = other RNA
ctttgcatgcatttgcactg

SEQ ID NO: 13929 - RNA, 20 nt, synthetic construct
  source 1..20: mol_type = other RNA
ttgcactgaggcgcgtgccc

SEQ ID NO: 13930 - RNA, 20 nt, synthetic construct
  source 1..20: mol_type = other RNA
actgaggcgcgtgcccaggt

SEQ ID NO: 13931 - RNA, 20 nt, synthetic construct
  source 1..20: mol_type = other RNA
ctgaggcgcgtgcccaggtc

SEQ ID NO: 13932 - RNA, 20 nt, synthetic construct
  source 1..20: mol_type = other RNA
tgaggcgcgtgcccaggtcg

SEQ ID NO: 13933 - RNA, 20 nt, synthetic construct
  source 1..20: mol_type = other RNA
gcgcgtgcccaggtcggggt

SEQ ID NO: 13934 - RNA, 20 nt, synthetic construct
  source 1..20: mol_type = other RNA
cccaggtcggggttggaaga

SEQ ID NO: 13935 - RNA, 20 nt, synthetic construct
  source 1..20: mol_type = other RNA
ccttcttccaaccccgacct

SEQ ID NO: 13936 - RNA, 20 nt, synthetic construct
  source 1..20: mol_type = other RNA
tccttcttccaaccccgacc

SEQ ID NO: 13937 - RNA, 20 nt, synthetic construct
  source 1..20: mol_type = other RNA
ggggttggaagaaggagagg

SEQ ID NO: 13938 - RNA, 20 nt, synthetic construct
  source 1..20: mol_type = other RNA
tgaaaggaaatgcttatgct

SEQ ID NO: 13939 - RNA, 20 nt, synthetic construct
  source 1..20: mol_type = other RNA
gggagagggaaaactctgaa

SEQ ID NO: 13940 - RNA, 20 nt, synthetic construct
  source 1..20: mol_type = other RNA
aaagggagagtttggggaga

SEQ ID NO: 13941 - RNA, 20 nt, synthetic construct
  source 1..20: mol_type = other RNA
aaaagggagagtttggggag

SEQ ID NO: 13942 - RNA, 20 nt, synthetic construct
  source 1..20: mol_type = other RNA
tgtgaaaaagggagagtttg

SEQ ID NO: 13943 - RNA, 20 nt, synthetic construct
  source 1..20: mol_type = other RNA
gtgtgaaaaagggagagttt

SEQ ID NO: 13944 - RNA, 20 nt, synthetic construct
  source 1..20: mol_type = other RNA
agtgtgaaaaagggagagtt

SEQ ID NO: 13945 - RNA, 20 nt, synthetic construct
  source 1..20: mol_type = other RNA
tttttcacactagtcaatac

SEQ ID NO: 13946 - RNA, 20 nt, synthetic construct
  source 1..20: mol_type = other RNA
ttttcacactagtcaataca

SEQ ID NO: 13947 - RNA, 20 nt, synthetic construct
  source 1..20: mol_type = other RNA
tttcacactagtcaatacag

SEQ ID NO: 13948 - RNA, 20 nt, synthetic construct
  source 1..20: mol_type = other RNA
tgtattgactagtgtgaaaa

SEQ ID NO: 13949 - RNA, 20 nt, synthetic construct
  source 1..20: mol_type = other RNA
tagtcaatacaggggtgtta

SEQ ID NO: 13950 - RNA, 20 nt, synthetic construct
  source 1..20: mol_type = other RNA
acaggggtgttaaggatgac

SEQ ID NO: 13951 - RNA, 20 nt, synthetic construct
  source 1..20: mol_type = other RNA
caggggtgttaaggatgact

SEQ ID NO: 13952 - RNA, 20 nt, synthetic construct
  source 1..20: mol_type = other RNA
aggggtgttaaggatgactg

SEQ ID NO: 13953 - RNA, 20 nt, synthetic construct
  source 1..20: mol_type = other RNA
tgttaaggatgactggggag

SEQ ID NO: 13954 - RNA, 20 nt, synthetic construct
  source 1..20: mol_type = other RNA
gttaaggatgactggggaga

SEQ ID NO: 13955 - RNA, 20 nt, synthetic construct
  source 1..20: mol_type = other RNA
ttaaggatgactggggagag

SEQ ID NO: 13956 - RNA, 20 nt, synthetic construct
  source 1..20: mol_type = other RNA
tgactggggagaggggaacg

SEQ ID NO: 13957 - RNA, 20 nt, synthetic construct
  source 1..20: mol_type = other RNA
ctggggagaggggaacgtgg

SEQ ID NO: 13958 - RNA, 20 nt, synthetic construct
  source 1..20: mol_type = other RNA
cgcgcgcagctgctctcctg

SEQ ID NO: 13959 - RNA, 20 nt, synthetic construct
  source 1..20: mol_type = other RNA
caggagagcagctgcgcgcg

SEQ ID NO: 13960 - RNA, 20 nt, synthetic construct
  source 1..20: mol_type = other RNA
tcaggagagcagctgcgcgc

SEQ ID NO: 13961 - RNA, 20 nt, synthetic construct
  source 1..20: mol_type = other RNA
ctcaggagagcagctgcgcg

SEQ ID NO: 13962 - RNA, 20 nt, synthetic construct
  source 1..20: mol_type = other RNA
gcagctgctctcctgaggct

SEQ ID NO: 13963 - RNA, 20 nt, synthetic construct
  source 1..20: mol_type = other RNA
cagctgctctcctgaggctc

SEQ ID NO: 13964 - RNA, 20 nt, synthetic construct
  source 1..20: mol_type = other RNA
tagtgcaggtcccgagcctc

SEQ ID NO: 13965 - RNA, 20 nt, synthetic construct
  source 1..20: mol_type = other RNA
gagaggggtggaggtagtgc

SEQ ID NO: 13966 - RNA, 20 nt, synthetic construct
  source 1..20: mol_type = other RNA
cctccacccctctcattccc

SEQ ID NO: 13967 - RNA, 20 nt, synthetic construct
  source 1..20: mol_type = other RNA
acccctctcattcccaggcc

SEQ ID NO: 13968 - RNA, 20 nt, synthetic construct
  source 1..20: mol_type = other RNA
aggcctgggaatgagagggg

SEQ ID NO: 13969 - RNA, 20 nt, synthetic construct
  source 1..20: mol_type = other RNA
gccaggcctgggaatgagag

SEQ ID NO: 13970 - RNA, 20 nt, synthetic construct
  source 1..20: mol_type = other RNA
agccaggcctgggaatgaga

SEQ ID NO: 13971 - RNA, 20 nt, synthetic construct
  source 1..20: mol_type = other RNA
gagccaggcctgggaatgag

SEQ ID NO: 13972 - RNA, 20 nt, synthetic construct
  source 1..20: mol_type = other RNA
gcgagggcggagccaggcct

SEQ ID NO: 13973 - RNA, 20 nt, synthetic construct
  source 1..20: mol_type = other RNA
ggcgagggcggagccaggcc

SEQ ID NO: 13974 - RNA, 20 nt, synthetic construct
  source 1..20: mol_type = other RNA
cggagggcgagggcggagcc

SEQ ID NO: 13975 - RNA, 20 nt, synthetic construct
  source 1..20: mol_type = other RNA
gggcgcgcggagggcgaggg

SEQ ID NO: 13976 - RNA, 20 nt, synthetic construct
  source 1..20: mol_type = other RNA
gccctccgcgcgcccgcttc

SEQ ID NO: 13977 - RNA, 20 nt, synthetic construct
  source 1..20: mol_type = other RNA
ccctccgcgcgcccgcttca

SEQ ID NO: 13978 - RNA, 20 nt, synthetic construct
  source 1..20: mol_type = other RNA
ccctgaagcgggcgcgcgga

SEQ ID NO: 13979 - RNA, 20 nt, synthetic construct
  source 1..20: mol_type = other RNA
gccctgaagcgggcgcgcgg

SEQ ID NO: 13980 - RNA, 20 nt, synthetic construct
  source 1..20: mol_type = other RNA
tcggccctgaagcgggcgcg

SEQ ID NO: 13981 - RNA, 20 nt, synthetic construct
  source 1..20: mol_type = other RNA
gcacttttcggccctgaagc

SEQ ID NO: 13982 - RNA, 20 nt, synthetic construct
  source 1..20: mol_type = other RNA
tgcacttttcggccctgaag

SEQ ID NO: 13983 - RNA, 20 nt, synthetic construct
  source 1..20: mol_type = other RNA
ggccgaaaagtgcattcctg

SEQ ID NO: 13984 - RNA, 20 nt, synthetic construct
  source 1..20: mol_type = other RNA
aaaagtgcattcctgcggct

SEQ ID NO: 13985 - RNA, 20 nt, synthetic construct
  source 1..20: mol_type = other RNA
agccgcaggaatgcactttt

SEQ ID NO: 13986 - RNA, 20 nt, synthetic construct
  source 1..20: mol_type = other RNA
ggcagcgcgcgccgagccgc

SEQ ID NO: 13987 - RNA, 20 nt, synthetic construct
  source 1..20: mol_type = other RNA
ggagacgggaaggaaggagg

SEQ ID NO: 13988 - RNA, 20 nt, synthetic construct
  source 1..20: mol_type = other RNA
tggggagacgggaaggaagg

SEQ ID NO: 13989 - RNA, 20 nt, synthetic construct
  source 1..20: mol_type = other RNA
ccttcccgtctccccacccg

SEQ ID NO: 13990 - RNA, 20 nt, synthetic construct
  source 1..20: mol_type = other RNA
gggtggggagacgggaagga

SEQ ID NO: 13991 - RNA, 20 nt, synthetic construct
  source 1..20: mol_type = other RNA
ccgcgggtggggagacggga

SEQ ID NO: 13992 - RNA, 20 nt, synthetic construct
  source 1..20: mol_type = other RNA
gtctccccacccgcggtcct

SEQ ID NO: 13993 - RNA, 20 nt, synthetic construct
  source 1..20: mol_type = other RNA
tctccccacccgcggtccta

SEQ ID NO: 13994 - RNA, 20 nt, synthetic construct
  source 1..20: mol_type = other RNA
aggaccgcgggtggggagac

SEQ ID NO: 13995 - RNA, 20 nt, synthetic construct
  source 1..20: mol_type = other RNA
taggaccgcgggtggggaga

SEQ ID NO: 13996 - RNA, 20 nt, synthetic construct
  source 1..20: mol_type = other RNA
cccacccgcggtcctagggc

SEQ ID NO: 13997 - RNA, 20 nt, synthetic construct
  source 1..20: mol_type = other RNA
cggccctaggaccgcgggtg

SEQ ID NO: 13998 - RNA, 20 nt, synthetic construct
  source 1..20: mol_type = other RNA
ccggccctaggaccgcgggt

SEQ ID NO: 13999 - RNA, 20 nt, synthetic construct
  source 1..20: mol_type = other RNA
tccggccctaggaccgcggg

SEQ ID NO: 14000 - RNA, 20 nt, synthetic construct
  source 1..20: mol_type = other RNA
cgctccggccctaggaccgc

SEQ ID NO: 14001 - RNA, 20 nt, synthetic construct
  source 1..20: mol_type = other RNA
gcgctccggccctaggaccg

SEQ ID NO: 14002 - RNA, 20 nt, synthetic construct
  source 1..20: mol_type = other RNA
cgggagcgcgctccggccct

SEQ ID NO: 14003 - RNA, 20 nt, synthetic construct
  source 1..20: mol_type = other RNA
ttcacggcgggagcgcgctc

SEQ ID NO: 14004 - RNA, 20 nt, synthetic construct
  source 1..20: mol_type = other RNA
cgctcccgccgtgaactctc

SEQ ID NO: 14005 - RNA, 20 nt, synthetic construct
  source 1..20: mol_type = other RNA
gctcccgccgtgaactctct

SEQ ID NO: 14006 - RNA, 20 nt, synthetic construct
  source 1..20: mol_type = other RNA
gttcccagagagttcacggc

SEQ ID NO: 14007 - RNA, 20 nt, synthetic construct
  source 1..20: mol_type = other RNA
ggttcccagagagttcacgg

SEQ ID NO: 14008 - RNA, 20 nt, synthetic construct
  source 1..20: mol_type = other RNA
aactctctgggaacccccct

SEQ ID NO: 14009 - RNA, 20 nt, synthetic construct
  source 1..20: mol_type = other RNA
actctctgggaacccccctc

SEQ ID NO: 14010 - RNA, 20 nt, synthetic construct
  source 1..20: mol_type = other RNA
ctctctgggaacccccctcg

SEQ ID NO: 14011 - RNA, 20 nt, synthetic construct
  source 1..20: mol_type = other RNA
tctgggaacccccctcgggg

SEQ ID NO: 14012 - RNA, 20 nt, synthetic construct
  source 1..20: mol_type = other RNA
ctgggaacccccctcggggc

SEQ ID NO: 14013 - RNA, 20 nt, synthetic construct
  source 1..20: mol_type = other RNA
ggaacccccctcggggcggg

SEQ ID NO: 14014 - RNA, 20 nt, synthetic construct
  source 1..20: mol_type = other RNA
tcggccacccgccccgaggg

SEQ ID NO: 14015 - RNA, 20 nt, synthetic construct
  source 1..20: mol_type = other RNA
ctcggccacccgccccgagg

SEQ ID NO: 14016 - RNA, 20 nt, synthetic construct
  source 1..20: mol_type = other RNA
gctcggccacccgccccgag

SEQ ID NO: 14017 - RNA, 20 nt, synthetic construct
  source 1..20: mol_type = other RNA
cgctcggccacccgccccga

SEQ ID NO: 14018 - RNA, 20 nt, synthetic construct
  source 1..20: mol_type = other RNA
gcgctcggccacccgccccg

SEQ ID NO: 14019 - RNA, 20 nt, synthetic construct
  source 1..20: mol_type = other RNA
caggaggaggtgagcgcgct

SEQ ID NO: 14020 - RNA, 20 nt, synthetic construct
  source 1..20: mol_type = other RNA
gcgctcacctcctcctgacc

SEQ ID NO: 14021 - RNA, 20 nt, synthetic construct
  source 1..20: mol_type = other RNA
ggcggggccgggtcaggagg

SEQ ID NO: 14022 - RNA, 20 nt, synthetic construct
  source 1..20: mol_type = other RNA
tggggcggggccgggtcagg

SEQ ID NO: 14023 - RNA, 20 nt, synthetic construct
  source 1..20: mol_type = other RNA
gggtggggcggggccgggtc

SEQ ID NO: 14024 - RNA, 20 nt, synthetic construct
  source 1..20: mol_type = other RNA
ggccccgccccaccccgccc

SEQ ID NO: 14025 - RNA, 20 nt, synthetic construct
  source 1..20: mol_type = other RNA
gggcggggtggggcggggcc

SEQ ID NO: 14026 - RNA, 20 nt, synthetic construct
  source 1..20: mol_type = other RNA
tgggcggggtggggcggggc

SEQ ID NO: 14027 - RNA, 20 nt, synthetic construct
  source 1..20: mol_type = other RNA
ggcctgggcggggtggggcg

SEQ ID NO: 14028 - RNA, 20 nt, synthetic construct
  source 1..20: mol_type = other RNA
cggcctgggcggggtggggc

SEQ ID NO: 14029 - RNA, 20 nt, synthetic construct
  source 1..20: mol_type = other RNA
acggcctgggcggggtgggg

SEQ ID NO: 14030 - RNA, 20 nt, synthetic construct
  source 1..20: mol_type = other RNA
aagacggcctgggcggggtg

SEQ ID NO: 14031 - RNA, 20 nt, synthetic construct
  source 1..20: mol_type = other RNA
gaagacggcctgggcggggt

SEQ ID NO: 14032 - RNA, 20 nt, synthetic construct
  source 1..20: mol_type = other RNA
tgaagacggcctgggcgggg

SEQ ID NO: 14033 - RNA, 20 nt, synthetic construct
  source 1..20: mol_type = other RNA
cgctgaagacggcctgggcg

SEQ ID NO: 14034 - RNA, 20 nt, synthetic construct
  source 1..20: mol_type = other RNA
gcgctgaagacggcctgggc

SEQ ID NO: 14035 - RNA, 20 nt, synthetic construct
  source 1..20: mol_type = other RNA
agcgctgaagacggcctggg

SEQ ID NO: 14036 - RNA, 20 nt, synthetic construct
  source 1..20: mol_type = other RNA
ggccgtcttcagcgctgccg

SEQ ID NO: 14037 - RNA, 20 nt, synthetic construct
  source 1..20: mol_type = other RNA
ggcagcgctgaagacggcct

SEQ ID NO: 14038 - RNA, 20 nt, synthetic construct
  source 1..20: mol_type = other RNA
cggcagcgctgaagacggcc

SEQ ID NO: 14039 - RNA, 20 nt, synthetic construct
  source 1..20: mol_type = other RNA
ctccgcggcagcgctgaaga

SEQ ID NO: 14040 - RNA, 20 nt, synthetic construct
  source 1..20: mol_type = other RNA
gagggggcggggggactccg

SEQ ID NO: 14041 - RNA, 20 nt, synthetic construct
  source 1..20: mol_type = other RNA
gctgcgctggagggggcggg

SEQ ID NO: 14042 - RNA, 20 nt, synthetic construct
  source 1..20: mol_type = other RNA
ggctgcgctggagggggcgg

SEQ ID NO: 14043 - RNA, 20 nt, synthetic construct
  source 1..20: mol_type = other RNA
tggctgcgctggagggggcg

SEQ ID NO: 14044 - RNA, 20 nt, synthetic construct
  source 1..20: mol_type = other RNA
ctggctgcgctggagggggc

SEQ ID NO: 14045 - RNA, 20 nt, synthetic construct
  source 1..20: mol_type = other RNA
tctggctgcgctggaggggg

SEQ ID NO: 14046 - RNA, 20 nt, synthetic construct
  source 1..20: mol_type = other RNA
gactctggctgcgctggagg

SEQ ID NO: 14047 - RNA, 20 nt, synthetic construct
  source 1..20: mol_type = other RNA
agactctggctgcgctggag

SEQ ID NO: 14048 - RNA, 20 nt, synthetic construct
  source 1..20: mol_type = other RNA
tagactctggctgcgctgga

SEQ ID NO: 14049 - RNA, 20 nt, synthetic construct
  source 1..20: mol_type = other RNA
gtagactctggctgcgctgg

SEQ ID NO: 14050 - RNA, 20 nt, synthetic construct
  source 1..20: mol_type = other RNA
ggggtagactctggctgcgc

SEQ ID NO: 14051 - RNA, 20 nt, synthetic construct
  source 1..20: mol_type = other RNA
gggctaggaggggtagactc

SEQ ID NO: 14052 - RNA, 20 nt, synthetic construct
  source 1..20: mol_type = other RNA
cggactgctcgggctaggag

SEQ ID NO: 14053 - RNA, 20 nt, synthetic construct
  source 1..20: mol_type = other RNA
gcggactgctcgggctagga

SEQ ID NO: 14054 - RNA, 20 nt, synthetic construct
  source 1..20: mol_type = other RNA
ggcggactgctcgggctagg

SEQ ID NO: 14055 - RNA, 20 nt, synthetic construct
  source 1..20: mol_type = other RNA
gagggcggactgctcgggct

SEQ ID NO: 14056 - RNA, 20 nt, synthetic construct
  source 1..20: mol_type = other RNA
gagcagtccgccctccgccg

SEQ ID NO: 14057 - RNA, 20 nt, synthetic construct
  source 1..20: mol_type = other RNA
cggcggagggcggactgctc

SEQ ID NO: 14058 - RNA, 20 nt, synthetic construct
  source 1..20: mol_type = other RNA
gcggcggagggcggactgct

SEQ ID NO: 14059 - RNA, 20 nt, synthetic construct
  source 1..20: mol_type = other RNA
gtccgccctccgccgcggcc

SEQ ID NO: 14060 - RNA, 20 nt, synthetic construct
  source 1..20: mol_type = other RNA
tccgccctccgccgcggccc

SEQ ID NO: 14061 - RNA, 20 nt, synthetic construct
  source 1..20: mol_type = other RNA
gcccgggccgcggcggaggg

SEQ ID NO: 14062 - RNA, 20 nt, synthetic construct
  source 1..20: mol_type = other RNA
gcggcccgggccgcggcgga

SEQ ID NO: 14063 - RNA, 20 nt, synthetic construct
  source 1..20: mol_type = other RNA
ggcggcccgggccgcggcgg

SEQ ID NO: 14064 - RNA, 20 nt, synthetic construct
  source 1..20: mol_type = other RNA
ggaggcggcccgggccgcgg

SEQ ID NO: 14065 - RNA, 20 nt, synthetic construct
  source 1..20: mol_type = other RNA
gagggaggcggcccgggccg

SEQ ID NO: 14066 - RNA, 20 nt, synthetic construct
  source 1..20: mol_type = other RNA
gactcggagggaggcggccc

SEQ ID NO: 14067 - RNA, 20 nt, synthetic construct
  source 1..20: mol_type = other RNA
ggactcggagggaggcggcc

SEQ ID NO: 14068 - RNA, 20 nt, synthetic construct
  source 1..20: mol_type = other RNA
ttcggggactcggagggagg

SEQ ID NO: 14069 - RNA, 20 nt, synthetic construct
  source 1..20: mol_type = other RNA
ggcttcggggactcggaggg

SEQ ID NO: 14070 - RNA, 20 nt, synthetic construct
  source 1..20: mol_type = other RNA
taaggcttcggggactcgga

SEQ ID NO: 14071 - RNA, 20 nt, synthetic construct
  source 1..20: mol_type = other RNA
ataaggcttcggggactcgg

SEQ ID NO: 14072 - RNA, 20 nt, synthetic construct
  source 1..20: mol_type = other RNA
gggataaggcttcggggact

SEQ ID NO: 14073 - RNA, 20 nt, synthetic construct
  source 1..20: mol_type = other RNA
agttgcgggataaggcttcg

SEQ ID NO: 14074 - RNA, 20 nt, synthetic construct
  source 1..20: mol_type = other RNA
cagttgcgggataaggcttc

SEQ ID NO: 14075 - RNA, 20 nt, synthetic construct
  source 1..20: mol_type = other RNA
tcagttgcgggataaggctt

SEQ ID NO: 14076 - RNA, 20 nt, synthetic construct
  source 1..20: mol_type = other RNA
ggggcgtcagttgcgggata

SEQ ID NO: 14077 - RNA, 20 nt, synthetic construct
  source 1..20: mol_type = other RNA
gcttagggggcgtcagttgc

SEQ ID NO: 14078 - RNA, 20 nt, synthetic construct
  source 1..20: mol_type = other RNA
cgcttagggggcgtcagttg

SEQ ID NO: 14079 - RNA, 20 nt, synthetic construct
  source 1..20: mol_type = other RNA
agacggtcgaggcgcttagg

SEQ ID NO: 14080 - RNA, 20 nt, synthetic construct
  source 1..20: mol_type = other RNA
gagacggtcgaggcgcttag

SEQ ID NO: 14081 - RNA, 20 nt, synthetic construct
  source 1..20: mol_type = other RNA
agagacggtcgaggcgctta

SEQ ID NO: 14082 - RNA, 20 nt, synthetic construct
  source 1..20: mol_type = other RNA
gagagacggtcgaggcgctt

SEQ ID NO: 14083 - RNA, 20 nt, synthetic construct
  source 1..20: mol_type = other RNA
agcatcgagagagacggtcg

SEQ ID NO: 14084 - RNA, 20 nt, synthetic construct
  source 1..20: mol_type = other RNA
agaaggagcatcgagagaga

SEQ ID NO: 14085 - RNA, 20 nt, synthetic construct
  source 1..20: mol_type = other RNA
agtgaagttatgttcgaaga

SEQ ID NO: 14086 - RNA, 20 nt, synthetic construct
  source 1..20: mol_type = other RNA
cacggcaggcacagcttatg

SEQ ID NO: 14087 - RNA, 20 nt, synthetic construct
  source 1..20: mol_type = other RNA
gcacggcaggcacagcttat

SEQ ID NO: 14088 - RNA, 20 nt, synthetic construct
  source 1..20: mol_type = other RNA
ggcacggcaggcacagctta

SEQ ID NO: 14089 - RNA, 20 nt, synthetic construct
  source 1..20: mol_type = other RNA
cgaggcgcagttggcacggc

SEQ ID NO: 14090 - RNA, 20 nt, synthetic construct
  source 1..20: mol_type = other RNA
tcatcgaggcgcagttggca

SEQ ID NO: 14091 - RNA, 20 nt, synthetic construct
  source 1..20: mol_type = other RNA
cagattcatcgaggcgcagt

SEQ ID NO: 14092 - RNA, 20 nt, synthetic construct
  source 1..20: mol_type = other RNA
ctcgatgaatctgcccctga

SEQ ID NO: 14093 - RNA, 20 nt, synthetic construct
  source 1..20: mol_type = other RNA
catcaggggcagattcatcg

SEQ ID NO: 14094 - RNA, 20 nt, synthetic construct
  source 1..20: mol_type = other RNA
ggaggggagttggccatcag

SEQ ID NO: 14095 - RNA, 20 nt, synthetic construct
  source 1..20: mol_type = other RNA
aggaggggagttggccatca

SEQ ID NO: 14096 - RNA, 20 nt, synthetic construct
  source 1..20: mol_type = other RNA
gaggaggggagttggccatc

SEQ ID NO: 14097 - RNA, 20 nt, synthetic construct
  source 1..20: mol_type = other RNA
agaaactggaggaggggagt

SEQ ID NO: 14098 - RNA, 20 nt, synthetic construct
  source 1..20: mol_type = other RNA
gcagtgagaaactggaggag

SEQ ID NO: 14099 - RNA, 20 nt, synthetic construct
  source 1..20: mol_type = other RNA
ggcagtgagaaactggagga

SEQ ID NO: 14100 - RNA, 20 nt, synthetic construct
  source 1..20: mol_type = other RNA
tggcagtgagaaactggagg

SEQ ID NO: 14101 - RNA, 20 nt, synthetic construct
  source 1..20: mol_type = other RNA
ccttggcagtgagaaactgg

SEQ ID NO: 14102 - RNA, 20 nt, synthetic construct
  source 1..20: mol_type = other RNA
agcccttggcagtgagaaac

SEQ ID NO: 14103 - RNA, 20 nt, synthetic construct
  source 1..20: mol_type = other RNA
ctcactgccaagggctccct

SEQ ID NO: 14104 - RNA, 20 nt, synthetic construct
  source 1..20: mol_type = other RNA
ccaagggctccctcggcaat

SEQ ID NO: 14105 - RNA, 20 nt, synthetic construct
  source 1..20: mol_type = other RNA
caagggctccctcggcaata

SEQ ID NO: 14106 - RNA, 20 nt, synthetic construct
  source 1..20: mol_type = other RNA
aagggctccctcggcaatag

SEQ ID NO: 14107 - RNA, 20 nt, synthetic construct
  source 1..20: mol_type = other RNA
cctattgccgagggagccct

SEQ ID NO: 14108 - RNA, 20 nt, synthetic construct
  source 1..20: mol_type = other RNA
ctcggcaataggggcgcttc

SEQ ID NO: 14109 - RNA, 20 nt, synthetic construct
  source 1..20: mol_type = other RNA
agaagcgcccctattgccga

SEQ ID NO: 14110 - RNA, 20 nt, synthetic construct
  source 1..20: mol_type = other RNA
cagaagcgcccctattgccg

SEQ ID NO: 14111 - RNA, 20 nt, synthetic construct
  source 1..20: mol_type = other RNA
tctggtcactgactgttctc

SEQ ID NO: 14112 - RNA, 20 nt, synthetic construct
  source 1..20: mol_type = other RNA
ctggtcactgactgttctca

SEQ ID NO: 14113 - RNA, 20 nt, synthetic construct
  source 1..20: mol_type = other RNA
ctttaaataccctctagcct

SEQ ID NO: 14114 - RNA, 20 nt, synthetic construct
  source 1..20: mol_type = other RNA
gcagttatgcctaggctaga

SEQ ID NO: 14115 - RNA, 20 nt, synthetic construct
  source 1..20: mol_type = other RNA
ggcagttatgcctaggctag

SEQ ID NO: 14116 - RNA, 20 nt, synthetic construct
  source 1..20: mol_type = other RNA
aggcataactgccctccctt

SEQ ID NO: 14117 - RNA, 20 nt, synthetic construct
  source 1..20: mol_type = other RNA
aagggagggcagttatgcct

SEQ ID NO: 14118 - RNA, 20 nt, synthetic construct
  source 1..20: mol_type = other RNA
aggggcactaaccgaaggga

SEQ ID NO: 14119 - RNA, 20 nt, synthetic construct
  source 1..20: mol_type = other RNA
gaggggcactaaccgaaggg

SEQ ID NO: 14120 - RNA, 20 nt, synthetic construct
  source 1..20: mol_type = other RNA
gctgaggggcactaaccgaa

SEQ ID NO: 14121 - RNA, 20 nt, synthetic construct
  source 1..20: mol_type = other RNA
agctgaggggcactaaccga

SEQ ID NO: 14122 - RNA, 20 nt, synthetic construct
  source 1..20: mol_type = other RNA
tagtgcccctcagctctcca

SEQ ID NO: 14123 - RNA, 20 nt, synthetic construct
  source 1..20: mol_type = other RNA
tgcggccttggagagctgag

SEQ ID NO: 14124 - RNA, 20 nt, synthetic construct
  source 1..20: mol_type = other RNA
ttgcggccttggagagctga

SEQ ID NO: 14125 - RNA, 20 nt, synthetic construct
  source 1..20: mol_type = other RNA
gttgcggccttggagagctg

SEQ ID NO: 14126 - RNA, 20 nt, synthetic construct
  source 1..20: mol_type = other RNA
aaggccgcaacactgttccc

SEQ ID NO: 14127 - RNA, 20 nt, synthetic construct
  source 1..20: mol_type = other RNA
aggccgcaacactgttccct

SEQ ID NO: 14128 - RNA, 20 nt, synthetic construct
  source 1..20: mol_type = other RNA
agggaacagtgttgcggcct

SEQ ID NO: 14129 - RNA, 20 nt, synthetic construct
  source 1..20: mol_type = other RNA
caacccagggaacagtgttg

SEQ ID NO: 14130 - RNA, 20 nt, synthetic construct
  source 1..20: mol_type = other RNA
gttccctgggttgccccttc

SEQ ID NO: 14131 - RNA, 20 nt, synthetic construct
  source 1..20: mol_type = other RNA
gtgccggaaggggcaaccca

SEQ ID NO: 14132 - RNA, 20 nt, synthetic construct
  source 1..20: mol_type = other RNA
agtgccggaaggggcaaccc

SEQ ID NO: 14133 - RNA, 20 nt, synthetic construct
  source 1..20: mol_type = other RNA
agggcgctcagtgccggaag

SEQ ID NO: 14134 - RNA, 20 nt, synthetic construct
  source 1..20: mol_type = other RNA
gagggcgctcagtgccggaa

SEQ ID NO: 14135 - RNA, 20 nt, synthetic construct
  source 1..20: mol_type = other RNA
cgagggcgctcagtgccgga

SEQ ID NO: 14136 - RNA, 20 nt, synthetic construct
  source 1..20: mol_type = other RNA
cactgagcgccctcgcccgg

SEQ ID NO: 14137 - RNA, 20 nt, synthetic construct
  source 1..20: mol_type = other RNA
cgggcgagggcgctcagtgc

SEQ ID NO: 14138 - RNA, 20 nt, synthetic construct
  source 1..20: mol_type = other RNA
gcgccctcgcccggcggaga

SEQ ID NO: 14139 - RNA, 20 nt, synthetic construct
  source 1..20: mol_type = other RNA
cgccctcgcccggcggagaa

SEQ ID NO: 14140 - RNA, 20 nt, synthetic construct
  source 1..20: mol_type = other RNA
gccctcgcccggcggagaag

SEQ ID NO: 14141 - RNA, 20 nt, synthetic construct
  source 1..20: mol_type = other RNA
ccctcgcccggcggagaagg

SEQ ID NO: 14142 - RNA, 20 nt, synthetic construct
  source 1..20: mol_type = other RNA
gcccggcggagaagggggtg

SEQ ID NO: 14143 - RNA, 20 nt, synthetic construct
  source 1..20: mol_type = other RNA
acccccttctccgccgggcg

SEQ ID NO: 14144 - RNA, 20 nt, synthetic construct
  source 1..20: mol_type = other RNA
cggcggagaagggggtgagg

SEQ ID NO: 14145 - RNA, 20 nt, synthetic construct
  source 1..20: mol_type = other RNA
ggcggagaagggggtgaggt

SEQ ID NO: 14146 - RNA, 20 nt, synthetic construct
  source 1..20: mol_type = other RNA
acctcacccccttctccgcc

SEQ ID NO: 14147 - RNA, 20 nt, synthetic construct
  source 1..20: mol_type = other RNA
ggagaagggggtgaggtggg

SEQ ID NO: 14148 - RNA, 20 nt, synthetic construct
  source 1..20: mol_type = other RNA
gagaagggggtgaggtgggc

SEQ ID NO: 14149 - RNA, 20 nt, synthetic construct
  source 1..20: mol_type = other RNA
agaagggggtgaggtgggcg

SEQ ID NO: 14150 - RNA, 20 nt, synthetic construct
  source 1..20: mol_type = other RNA
gaagggggtgaggtgggcgg

SEQ ID NO: 14151 - RNA, 20 nt, synthetic construct
  source 1..20: mol_type = other RNA
aagggggtgaggtgggcggg

SEQ ID NO: 14152 - RNA, 20 nt, synthetic construct
  source 1..20: mol_type = other RNA
gggtgaggtgggcggggggc

SEQ ID NO: 14153 - RNA, 20 nt, synthetic construct
  source 1..20: mol_type = other RNA
gccacgtcagaagtttgccc

SEQ ID NO: 14154 - RNA, 20 nt, synthetic construct
  source 1..20: mol_type = other RNA
gtcagaagtttgccctggcc

SEQ ID NO: 14155 - RNA, 20 nt, synthetic construct
  source 1..20: mol_type = other RNA
gccagggcaaacttctgacg

SEQ ID NO: 14156 - RNA, 20 nt, synthetic construct
  source 1..20: mol_type = other RNA
gaagtttgccctggcccggc

SEQ ID NO: 14157 - RNA, 20 nt, synthetic construct
  source 1..20: mol_type = other RNA
aagtttgccctggcccggca

SEQ ID NO: 14158 - RNA, 20 nt, synthetic construct
  source 1..20: mol_type = other RNA
cctggcccggcagggccgaa

SEQ ID NO: 14159 - RNA, 20 nt, synthetic construct
  source 1..20: mol_type = other RNA
ctggcccggcagggccgaat

SEQ ID NO: 14160 - RNA, 20 nt, synthetic construct
  source 1..20: mol_type = other RNA
tggcccggcagggccgaatg

SEQ ID NO: 14161 - RNA, 20 nt, synthetic construct
  source 1..20: mol_type = other RNA
ggcccggcagggccgaatgg

SEQ ID NO: 14162 - RNA, 20 nt, synthetic construct
  source 1..20: mol_type = other RNA
cattcggccctgccgggcca

SEQ ID NO: 14163 - RNA, 20 nt, synthetic construct
  source 1..20: mol_type = other RNA
ccattcggccctgccgggcc

SEQ ID NO: 14164 - RNA, 20 nt, synthetic construct
  source 1..20: mol_type = other RNA
tccccccattcggccctgcc

SEQ ID NO: 14165 - RNA, 20 nt, synthetic construct
  source 1..20: mol_type = other RNA
gtccccccattcggccctgc

SEQ ID NO: 14166 - RNA, 20 nt, synthetic construct
  source 1..20: mol_type = other RNA
gaatggggggaccctggccc

SEQ ID NO: 14167 - RNA, 20 nt, synthetic construct
  source 1..20: mol_type = other RNA
ggggccagggtccccccatt

SEQ ID NO: 14168 - RNA, 20 nt, synthetic construct
  source 1..20: mol_type = other RNA
gctggcgctgtccggggcca

SEQ ID NO: 14169 - RNA, 20 nt, synthetic construct
  source 1..20: mol_type = other RNA
tgctggcgctgtccggggcc

SEQ ID NO: 14170 - RNA, 20 nt, synthetic construct
  source 1..20: mol_type = other RNA
gccgctgctggcgctgtccg

SEQ ID NO: 14171 - RNA, 20 nt, synthetic construct
  source 1..20: mol_type = other RNA
cgccgctgctggcgctgtcc

SEQ ID NO: 14172 - RNA, 20 nt, synthetic construct
  source 1..20: mol_type = other RNA
tcgccgctgctggcgctgtc

SEQ ID NO: 14173 - RNA, 20 nt, synthetic construct
  source 1..20: mol_type = other RNA
gcgccagcagcggcgactcc

SEQ ID NO: 14174 - RNA, 20 nt, synthetic construct
  source 1..20: mol_type = other RNA
tttccgggagtcgccgctgc

SEQ ID NO: 14175 - RNA, 20 nt, synthetic construct
  source 1..20: mol_type = other RNA
cgggggagggggggatttcc

SEQ ID NO: 14176 - RNA, 20 nt, synthetic construct
  source 1..20: mol_type = other RNA
gcgggggagggggggatttc

SEQ ID NO: 14177 - RNA, 20 nt, synthetic construct
  source 1..20: mol_type = other RNA
ggcggggcgcgggggagggg

SEQ ID NO: 14178 - RNA, 20 nt, synthetic construct
  source 1..20: mol_type = other RNA
gggcggggcgcgggggaggg

SEQ ID NO: 14179 - RNA, 20 nt, synthetic construct
  source 1..20: mol_type = other RNA
agggcggggcgcgggggagg

SEQ ID NO: 14180 - RNA, 20 nt, synthetic construct
  source 1..20: mol_type = other RNA
gagggcggggcgcgggggag

SEQ ID NO: 14181 - RNA, 20 nt, synthetic construct
  source 1..20: mol_type = other RNA
tgagggcggggcgcggggga

SEQ ID NO: 14182 - RNA, 20 nt, synthetic construct
  source 1..20: mol_type = other RNA
ctgagggcggggcgcggggg

SEQ ID NO: 14183 - RNA, 20 nt, synthetic construct
  source 1..20: mol_type = other RNA
cgcgccccgccctcagccgc

SEQ ID NO: 14184 - RNA, 20 nt, synthetic construct
  source 1..20: mol_type = other RNA
gcgccccgccctcagccgcc

SEQ ID NO: 14185 - RNA, 20 nt, synthetic construct
  source 1..20: mol_type = other RNA
gcggctgagggcggggcgcg

SEQ ID NO: 14186 - RNA, 20 nt, synthetic construct
  source 1..20: mol_type = other RNA
ggcggctgagggcggggcgc

SEQ ID NO: 14187 - RNA, 20 nt, synthetic construct
  source 1..20: mol_type = other RNA
cggcggctgagggcggggcg

SEQ ID NO: 14188 - RNA, 20 nt, synthetic construct
  source 1..20: mol_type = other RNA
ccctcagccgccgggccgcc

SEQ ID NO: 14189 - RNA, 20 nt, synthetic construct
  source 1..20: mol_type = other RNA
gcggcccggcggctgagggc

SEQ ID NO: 14190 - RNA, 20 nt, synthetic construct
  source 1..20: mol_type = other RNA
ggcggcccggcggctgaggg

SEQ ID NO: 14191 - RNA, 20 nt, synthetic construct
  source 1..20: mol_type = other RNA
ccgggcggcccggcggctga

SEQ ID NO: 14192 - RNA, 20 nt, synthetic construct
  source 1..20: mol_type = other RNA
gccgggcggcccggcggctg

SEQ ID NO: 14193 - RNA, 20 nt, synthetic construct
  source 1..20: mol_type = other RNA
aggcaggccgggcggcccgg

SEQ ID NO: 14194 - RNA, 20 nt, synthetic construct
  source 1..20: mol_type = other RNA
ggcaggcaggccgggcggcc

SEQ ID NO: 14195 - RNA, 20 nt, synthetic construct
  source 1..20: mol_type = other RNA
gcccggcctgcctgcccagc

SEQ ID NO: 14196 - RNA, 20 nt, synthetic construct
  source 1..20: mol_type = other RNA
ggctgggcaggcaggccggg

SEQ ID NO: 14197 - RNA, 20 nt, synthetic construct
  source 1..20: mol_type = other RNA
gccggctgggcaggcaggcc

SEQ ID NO: 14198 - RNA, 20 nt, synthetic construct
  source 1..20: mol_type = other RNA
agccggctgggcaggcaggc

SEQ ID NO: 14199 - RNA, 20 nt, synthetic construct
  source 1..20: mol_type = other RNA
acagagccggctgggcaggc

SEQ ID NO: 14200 - RNA, 20 nt, synthetic construct
  source 1..20: mol_type = other RNA
gctgacagagccggctgggc

SEQ ID NO: 14201 - RNA, 20 nt, synthetic construct
  source 1..20: mol_type = other RNA
cggcgctgacagagccggct

SEQ ID NO: 14202 - RNA, 20 nt, synthetic construct
  source 1..20: mol_type = other RNA
gcggcgctgacagagccggc

SEQ ID NO: 14203 - RNA, 20 nt, synthetic construct
  source 1..20: mol_type = other RNA
ctctgtcagcgccgctcaca

SEQ ID NO: 14204 - RNA, 20 nt, synthetic construct
  source 1..20: mol_type = other RNA
tctgtcagcgccgctcacac

SEQ ID NO: 14205 - RNA, 20 nt, synthetic construct
  source 1..20: mol_type = other RNA
cgctcacacgggcagcgccg

SEQ ID NO: 14206 - RNA, 20 nt, synthetic construct
  source 1..20: mol_type = other RNA
cgcggcgctgcccgtgtgag

SEQ ID NO: 14207 - RNA, 20 nt, synthetic construct
  source 1..20: mol_type = other RNA
acacgggcagcgccgcggag

SEQ ID NO: 14208 - RNA, 20 nt, synthetic construct
  source 1..20: mol_type = other RNA
cacgggcagcgccgcggagc

SEQ ID NO: 14209 - RNA, 20 nt, synthetic construct
  source 1..20: mol_type = other RNA
gcagcgccgcggagcgggag

SEQ ID NO: 14210 - RNA, 20 nt, synthetic construct
  source 1..20: mol_type = other RNA
cgcggagcgggagcggcgcc

SEQ ID NO: 14211 - RNA, 20 nt, synthetic construct
  source 1..20: mol_type = other RNA
cgggcgccgctcccgctccg

SEQ ID NO: 14212 - RNA, 20 nt, synthetic construct
  source 1..20: mol_type = other RNA
agcgggagcggcgcccggcc

SEQ ID NO: 14213 - RNA, 20 nt, synthetic construct
  source 1..20: mol_type = other RNA
ggcccggcccttcccccgcc

SEQ ID NO: 14214 - RNA, 20 nt, synthetic construct
  source 1..20: mol_type = other RNA
ggcgggggaagggccgggcc

SEQ ID NO: 14215 - RNA, 20 nt, synthetic construct
  source 1..20: mol_type = other RNA
tggcgggggaagggccgggc

SEQ ID NO: 14216 - RNA, 20 nt, synthetic construct
  source 1..20: mol_type = other RNA
cgcctggcgggggaagggcc

SEQ ID NO: 14217 - RNA, 20 nt, synthetic construct
  source 1..20: mol_type = other RNA
ccgcctggcgggggaagggc

SEQ ID NO: 14218 - RNA, 20 nt, synthetic construct
  source 1..20: mol_type = other RNA
cttcccccgccaggcggctg

SEQ ID NO: 14219 - RNA, 20 nt, synthetic construct
  source 1..20: mol_type = other RNA
acagccgcctggcgggggaa

SEQ ID NO: 14220 - RNA, 20 nt, synthetic construct
  source 1..20: mol_type = other RNA
cacagccgcctggcggggga

SEQ ID NO: 14221 - RNA, 20 nt, synthetic construct
  source 1..20: mol_type = other RNA
cccgccaggcggctgtggct

SEQ ID NO: 14222 - RNA, 20 nt, synthetic construct
  source 1..20: mol_type = other RNA
cagccacagccgcctggcgg

SEQ ID NO: 14223 - RNA, 20 nt, synthetic construct
  source 1..20: mol_type = other RNA
ccagccacagccgcctggcg

SEQ ID NO: 14224 - RNA, 20 nt, synthetic construct
  source 1..20: mol_type = other RNA
cccagccacagccgcctggc

SEQ ID NO: 14225 - RNA, 20 nt, synthetic construct
  source 1..20: mol_type = other RNA
gcccagccacagccgcctgg

SEQ ID NO: 14226 - RNA, 20 nt, synthetic construct
  source 1..20: mol_type = other RNA
ctggcccagccacagccgcc

SEQ ID NO: 14227 - RNA, 20 nt, synthetic construct
  source 1..20: mol_type = other RNA
ggctgtggctgggccagggc

SEQ ID NO: 14228 - RNA, 20 nt, synthetic construct
  source 1..20: mol_type = other RNA
gctgtggctgggccagggcg

SEQ ID NO: 14229 - RNA, 20 nt, synthetic construct
  source 1..20: mol_type = other RNA
gggacaggggtttggcctaa

SEQ ID NO: 14230 - RNA, 20 nt, synthetic construct
  source 1..20: mol_type = other RNA
gcaggcaggggacaggggtt

SEQ ID NO: 14231 - RNA, 20 nt, synthetic construct
  source 1..20: mol_type = other RNA
ggaaggcaggcaggggacag

SEQ ID NO: 14232 - RNA, 20 nt, synthetic construct
  source 1..20: mol_type = other RNA
aggaaggcaggcaggggaca

SEQ ID NO: 14233 - RNA, 20 nt, synthetic construct
  source 1..20: mol_type = other RNA
taggaaggcaggcaggggac

SEQ ID NO: 14234 - RNA, 20 nt, synthetic construct
  source 1..20: mol_type = other RNA
ccctgcctgccttcctaact

SEQ ID NO: 14235 - RNA, 20 nt, synthetic construct
  source 1..20: mol_type = other RNA
cctgcctgccttcctaactg

SEQ ID NO: 14236 - RNA, 20 nt, synthetic construct
  source 1..20: mol_type = other RNA
ccagttaggaaggcaggcag

SEQ ID NO: 14237 - RNA, 20 nt, synthetic construct
  source 1..20: mol_type = other RNA
cccagttaggaaggcaggca

SEQ ID NO: 14238 - RNA, 20 nt, synthetic construct
  source 1..20: mol_type = other RNA
ccccagttaggaaggcaggc

SEQ ID NO: 14239 - RNA, 20 nt, synthetic construct
  source 1..20: mol_type = other RNA
ggcaccccagttaggaaggc

SEQ ID NO: 14240 - RNA, 20 nt, synthetic construct
  source 1..20: mol_type = other RNA
agttggcaccccagttagga

SEQ ID NO: 14241 - RNA, 20 nt, synthetic construct
  source 1..20: mol_type = other RNA
aaagagttggcaccccagtt

SEQ ID NO: 14242 - RNA, 20 nt, synthetic construct
  source 1..20: mol_type = other RNA
agggtggatggtaaaagagt

SEQ ID NO: 14243 - RNA, 20 nt, synthetic construct
  source 1..20: mol_type = other RNA
gaaggcatcaggagggtgga

SEQ ID NO: 14244 - RNA, 20 nt, synthetic construct
  source 1..20: mol_type = other RNA
acaagaaggcatcaggaggg

SEQ ID NO: 14245 - RNA, 20 nt, synthetic construct
  source 1..20: mol_type = other RNA
ttaacaagaaggcatcagga

SEQ ID NO: 14246 - RNA, 20 nt, synthetic construct
  source 1..20: mol_type = other RNA
gttaacaagaaggcatcagg

SEQ ID NO: 14247 - RNA, 20 nt, synthetic construct
  source 1..20: mol_type = other RNA
aatgttaacaagaaggcatc

SEQ ID NO: 14248 - RNA, 20 nt, synthetic construct
  source 1..20: mol_type = other RNA
gaaggcaaatgttaacaaga

SEQ ID NO: 14249 - RNA, 20 nt, synthetic construct
  source 1..20: mol_type = other RNA
tcagggatcttggggaatga

SEQ ID NO: 14250 - RNA, 20 nt, synthetic construct
  source 1..20: mol_type = other RNA
tgtgagtctcagggatcttg

SEQ ID NO: 14251 - RNA, 20 nt, synthetic construct
  source 1..20: mol_type = other RNA
gtgtgagtctcagggatctt

SEQ ID NO: 14252 - RNA, 20 nt, synthetic construct
  source 1..20: mol_type = other RNA
tgtgtgagtctcagggatct

SEQ ID NO: 14253 - RNA, 20 nt, synthetic construct
  source 1..20: mol_type = other RNA
tccctgagactcacacagag

SEQ ID NO: 14254 - RNA, 20 nt, synthetic construct
  source 1..20: mol_type = other RNA
gcctctctgtgtgagtctca

SEQ ID NO: 14255 - RNA, 20 nt, synthetic construct
  source 1..20: mol_type = other RNA
ggcctctctgtgtgagtctc

SEQ ID NO: 14256 - RNA, 20 nt, synthetic construct
  source 1..20: mol_type = other RNA
acacagagaggccatctcct

SEQ ID NO: 14257 - RNA, 20 nt, synthetic construct
  source 1..20: mol_type = other RNA
cacagagaggccatctcctt

SEQ ID NO: 14258 - RNA, 20 nt, synthetic construct
  source 1..20: mol_type = other RNA
acagagaggccatctccttg

SEQ ID NO: 14259 - RNA, 20 nt, synthetic construct
  source 1..20: mol_type = other RNA
gagaggccatctccttgggg

SEQ ID NO: 14260 - RNA, 20 nt, synthetic construct
  source 1..20: mol_type = other RNA
gccatctccttggggaggtc

SEQ ID NO: 14261 - RNA, 20 nt, synthetic construct
  source 1..20: mol_type = other RNA
tctccttggggaggtcaggc

SEQ ID NO: 14262 - RNA, 20 nt, synthetic construct
  source 1..20: mol_type = other RNA
gcctgacctccccaaggaga

SEQ ID NO: 14263 - RNA, 20 nt, synthetic construct
  source 1..20: mol_type = other RNA
tggggaggtcaggctggccc

SEQ ID NO: 14264 - RNA, 20 nt, synthetic construct
  source 1..20: mol_type = other RNA
gggccagcctgacctcccca

SEQ ID NO: 14265 - RNA, 20 nt, synthetic construct
  source 1..20: mol_type = other RNA
ggtcaggctggcccaggccc

SEQ ID NO: 14266 - RNA, 20 nt, synthetic construct
  source 1..20: mol_type = other RNA
tggcccaggccccggaagct

SEQ ID NO: 14267 - RNA, 20 nt, synthetic construct
  source 1..20: mol_type = other RNA
ggcccaggccccggaagcta

SEQ ID NO: 14268 - RNA, 20 nt, synthetic construct
  source 1..20: mol_type = other RNA
agccctagcttccggggcct

SEQ ID NO: 14269 - RNA, 20 nt, synthetic construct
  source 1..20: mol_type = other RNA
gagccctagcttccggggcc

SEQ ID NO: 14270 - RNA, 20 nt, synthetic construct
  source 1..20: mol_type = other RNA
atgctgagccctagcttccg

SEQ ID NO: 14271 - RNA, 20 nt, synthetic construct
  source 1..20: mol_type = other RNA
gatgctgagccctagcttcc

SEQ ID NO: 14272 - RNA, 20 nt, synthetic construct
  source 1..20: mol_type = other RNA
agatgctgagccctagcttc

SEQ ID NO: 14273 - RNA, 20 nt, synthetic construct
  source 1..20: mol_type = other RNA
ctagggctcagcatctcgaa

SEQ ID NO: 14274 - RNA, 20 nt, synthetic construct
  source 1..20: mol_type = other RNA
gggctcagcatctcgaaagg

SEQ ID NO: 14275 - RNA, 20 nt, synthetic construct
  source 1..20: mol_type = other RNA
ggagaccccctgagtgcccc

SEQ ID NO: 14276 - RNA, 20 nt, synthetic construct
  source 1..20: mol_type = other RNA
gagaccccctgagtgcccct

SEQ ID NO: 14277 - RNA, 20 nt, synthetic construct
  source 1..20: mol_type = other RNA
ccccctgagtgcccctggga

SEQ ID NO: 14278 - RNA, 20 nt, synthetic construct
  source 1..20: mol_type = other RNA
ccttcccaggggcactcagg

SEQ ID NO: 14279 - RNA, 20 nt, synthetic construct
  source 1..20: mol_type = other RNA
gagtgcccctgggaaggcga

SEQ ID NO: 14280 - RNA, 20 nt, synthetic construct
  source 1..20: mol_type = other RNA
cgccttcccaggggcactca

SEQ ID NO: 14281 - RNA, 20 nt, synthetic construct
  source 1..20: mol_type = other RNA
tcgccttcccaggggcactc

SEQ ID NO: 14282 - RNA, 20 nt, synthetic construct
  source 1..20: mol_type = other RNA
tttccccttcgccttcccag

SEQ ID NO: 14283 - RNA, 20 nt, synthetic construct
  source 1..20: mol_type = other RNA
gtttccccttcgccttccca

SEQ ID NO: 14284 - RNA, 20 nt, synthetic construct
  source 1..20: mol_type = other RNA
ggtttccccttcgccttccc

SEQ ID NO: 14285 - RNA, 20 nt, synthetic construct
  source 1..20: mol_type = other RNA
gcgaaggggaaacctgcccc

SEQ ID NO: 14286 - RNA, 20 nt, synthetic construct
  source 1..20: mol_type = other RNA
cgaaggggaaacctgcccct

SEQ ID NO: 14287 - RNA, 20 nt, synthetic construct
  source 1..20: mol_type = other RNA
gcccctgggtagccagatcc

SEQ ID NO: 14288 - RNA, 20 nt, synthetic construct
  source 1..20: mol_type = other RNA
ggatctggctacccaggggc

SEQ ID NO: 14289 - RNA, 20 nt, synthetic construct
  source 1..20: mol_type = other RNA
gcctggatctggctacccag

SEQ ID NO: 14290 - RNA, 20 nt, synthetic construct
  source 1..20: mol_type = other RNA
ggcctggatctggctaccca

SEQ ID NO: 14291 - RNA, 20 nt, synthetic construct
  source 1..20: mol_type = other RNA
gtagccagatccaggcccca

SEQ ID NO: 14292 - RNA, 20 nt, synthetic construct
  source 1..20: mol_type = other RNA
ggtgccctggggcctggatc

SEQ ID NO: 14293 - RNA, 20 nt, synthetic construct
  source 1..20: mol_type = other RNA
gcggctggtgccctggggcc

SEQ ID NO: 14294 - RNA, 20 nt, synthetic construct
  source 1..20: mol_type = other RNA
tctttgcggctggtgccctg

SEQ ID NO: 14295 - RNA, 20 nt, synthetic construct
  source 1..20: mol_type = other RNA
ctctttgcggctggtgccct

SEQ ID NO: 14296 - RNA, 20 nt, synthetic construct
  source 1..20: mol_type = other RNA
actctttgcggctggtgccc

SEQ ID NO: 14297 - RNA, 20 nt, synthetic construct
  source 1..20: mol_type = other RNA
aaggagcgactctttgcggc

SEQ ID NO: 14298 - RNA, 20 nt, synthetic construct
  source 1..20: mol_type = other RNA
aaagagtcgctccttattgg

SEQ ID NO: 14299 - RNA, 20 nt, synthetic construct
  source 1..20: mol_type = other RNA
caataaggagcgactctttg

SEQ ID NO: 14300 - RNA, 20 nt, synthetic construct
  source 1..20: mol_type = other RNA
tcgctccttattggtggcca

SEQ ID NO: 14301 - RNA, 20 nt, synthetic construct
  source 1..20: mol_type = other RNA
attggtggccatggcagctg

SEQ ID NO: 14302 - RNA, 20 nt, synthetic construct
  source 1..20: mol_type = other RNA
agctgccatggccaccaata

SEQ ID NO: 14303 - RNA, 20 nt, synthetic construct
  source 1..20: mol_type = other RNA
ctctcacaccgcagctgcca

SEQ ID NO: 14304 - RNA, 20 nt, synthetic construct
  source 1..20: mol_type = other RNA
gctgcggtgtgagagtcccc

SEQ ID NO: 14305 - RNA, 20 nt, synthetic construct
  source 1..20: mol_type = other RNA
ctgcggtgtgagagtcccct

SEQ ID NO: 14306 - RNA, 20 nt, synthetic construct
  source 1..20: mol_type = other RNA
tgcggtgtgagagtcccctg

SEQ ID NO: 14307 - RNA, 20 nt, synthetic construct
  source 1..20: mol_type = other RNA
gagtcccctggggtctgcag

SEQ ID NO: 14308 - RNA, 20 nt, synthetic construct
  source 1..20: mol_type = other RNA
agtcccctggggtctgcagt

SEQ ID NO: 14309 - RNA, 20 nt, synthetic construct
  source 1..20: mol_type = other RNA
cccctggggtctgcagtggg

SEQ ID NO: 14310 - RNA, 20 nt, synthetic construct
  source 1..20: mol_type = other RNA
ccctggggtctgcagtgggc

SEQ ID NO: 14311 - RNA, 20 nt, synthetic construct
  source 1..20: mol_type = other RNA
ccgcccactgcagaccccag

SEQ ID NO: 14312 - RNA, 20 nt, synthetic construct
  source 1..20: mol_type = other RNA
gggtctgcagtgggcgggcg

SEQ ID NO: 14313 - RNA, 20 nt, synthetic construct
  source 1..20: mol_type = other RNA
gcccgcccactgcagacccc

SEQ ID NO: 14314 - RNA, 20 nt, synthetic construct
  source 1..20: mol_type = other RNA
gtgggcatgggcaggggctg

SEQ ID NO: 14315 - RNA, 20 nt, synthetic construct
  source 1..20: mol_type = other RNA
ggggcagtgggcatgggcag

SEQ ID NO: 14316 - RNA, 20 nt, synthetic construct
  source 1..20: mol_type = other RNA
tggggcagtgggcatgggca

SEQ ID NO: 14317 - RNA, 20 nt, synthetic construct
  source 1..20: mol_type = other RNA
ccatgcccactgccccagcc

SEQ ID NO: 14318 - RNA, 20 nt, synthetic construct
  source 1..20: mol_type = other RNA
catgcccactgccccagcct

SEQ ID NO: 14319 - RNA, 20 nt, synthetic construct
  source 1..20: mol_type = other RNA
caggctggggcagtgggcat

SEQ ID NO: 14320 - RNA, 20 nt, synthetic construct
  source 1..20: mol_type = other RNA
ccaggctggggcagtgggca

SEQ ID NO: 14321 - RNA, 20 nt, synthetic construct
  source 1..20: mol_type = other RNA
gcctcccaggctggggcagt

SEQ ID NO: 14322 - RNA, 20 nt, synthetic construct
  source 1..20: mol_type = other RNA
agcctcccaggctggggcag

SEQ ID NO: 14323 - RNA, 20 nt, synthetic construct
  source 1..20: mol_type = other RNA
gtacggagcctcccaggctg

SEQ ID NO: 14324 - RNA, 20 nt, synthetic construct
  source 1..20: mol_type = other RNA
ggtacggagcctcccaggct

SEQ ID NO: 14325 - RNA, 20 nt, synthetic construct
  source 1..20: mol_type = other RNA
gggtacggagcctcccaggc

SEQ ID NO: 14326 - RNA, 20 nt, synthetic construct
  source 1..20: mol_type = other RNA
gggcgggtacggagcctccc

SEQ ID NO: 14327 - RNA, 20 nt, synthetic construct
  source 1..20: mol_type = other RNA
ggctccgtacccgccctgcc

SEQ ID NO: 14328 - RNA, 20 nt, synthetic construct
  source 1..20: mol_type = other RNA
caggccaggcagggcgggta

SEQ ID NO: 14329 - RNA, 20 nt, synthetic construct
  source 1..20: mol_type = other RNA
gccctgcctggcctgcccac

SEQ ID NO: 14330 - RNA, 20 nt, synthetic construct
  source 1..20: mol_type = other RNA
ccctgcctggcctgcccact

SEQ ID NO: 14331 - RNA, 20 nt, synthetic construct
  source 1..20: mol_type = other RNA
gtgggcaggccaggcagggc

SEQ ID NO: 14332 - RNA, 20 nt, synthetic construct
  source 1..20: mol_type = other RNA
agtgggcaggccaggcaggg

SEQ ID NO: 14333 - RNA, 20 nt, synthetic construct
  source 1..20: mol_type = other RNA
cccagtgggcaggccaggca

SEQ ID NO: 14334 - RNA, 20 nt, synthetic construct
  source 1..20: mol_type = other RNA
gcccagtgggcaggccaggc

SEQ ID NO: 14335 - RNA, 20 nt, synthetic construct
  source 1..20: mol_type = other RNA
ggaggcccagtgggcaggcc

SEQ ID NO: 14336 - RNA, 20 nt, synthetic construct
  source 1..20: mol_type = other RNA
cttttggaggcccagtgggc

SEQ ID NO: 14337 - RNA, 20 nt, synthetic construct
  source 1..20: mol_type = other RNA
actgggcctccaaaagtcct

SEQ ID NO: 14338 - RNA, 20 nt, synthetic construct
  source 1..20: mol_type = other RNA
ctgggcctccaaaagtccta

SEQ ID NO: 14339 - RNA, 20 nt, synthetic construct
  source 1..20: mol_type = other RNA
aggacttttggaggcccagt

SEQ ID NO: 14340 - RNA, 20 nt, synthetic construct
  source 1..20: mol_type = other RNA
taggacttttggaggcccag

SEQ ID NO: 14341 - RNA, 20 nt, synthetic construct
  source 1..20: mol_type = other RNA
tttctccctaggacttttgg

SEQ ID NO: 14342 - RNA, 20 nt, synthetic construct
  source 1..20: mol_type = other RNA
ctctttctccctaggacttt

SEQ ID NO: 14343 - RNA, 20 nt, synthetic construct
  source 1..20: mol_type = other RNA
ctagggagaaagagagagaa

SEQ ID NO: 14344 - RNA, 20 nt, synthetic construct
  source 1..20: mol_type = other RNA
ctttctctctctttctccct

SEQ ID NO: 14345 - RNA, 20 nt, synthetic construct
  source 1..20: mol_type = other RNA
atgagagaatgaccactctg

SEQ ID NO: 14346 - RNA, 20 nt, synthetic construct
  source 1..20: mol_type = other RNA
cagggcttggaacctcagag

SEQ ID NO: 14347 - RNA, 20 nt, synthetic construct
  source 1..20: mol_type = other RNA
tgagagagggtcacagggct

SEQ ID NO: 14348 - RNA, 20 nt, synthetic construct
  source 1..20: mol_type = other RNA
gcaactgagagagggtcaca

SEQ ID NO: 14349 - RNA, 20 nt, synthetic construct
  source 1..20: mol_type = other RNA
tgcaactgagagagggtcac

SEQ ID NO: 14350 - RNA, 20 nt, synthetic construct
  source 1..20: mol_type = other RNA
agaagactgcaactgagaga

SEQ ID NO: 14351 - RNA, 20 nt, synthetic construct
  source 1..20: mol_type = other RNA
gagaagactgcaactgagag

SEQ ID NO: 14352 - RNA, 20 nt, synthetic construct
  source 1..20: mol_type = other RNA
ataaactgtagcagcacaga

SEQ ID NO: 14353 - RNA, 20 nt, synthetic construct
  source 1..20: mol_type = other RNA
gataaactgtagcagcacag

SEQ ID NO: 14354 - RNA, 20 nt, synthetic construct
  source 1..20: mol_type = other RNA
tgctacagtttatcctgccc

SEQ ID NO: 14355 - RNA, 20 nt, synthetic construct
  source 1..20: mol_type = other RNA
agtttatcctgccctggctc

SEQ ID NO: 14356 - RNA, 20 nt, synthetic construct
  source 1..20: mol_type = other RNA
gggctctggtcctgggcagc

SEQ ID NO: 14357 - RNA, 20 nt, synthetic construct
  source 1..20: mol_type = other RNA
ccaggaccagagccctaaag

SEQ ID NO: 14358 - RNA, 20 nt, synthetic construct
  source 1..20: mol_type = other RNA
caggaccagagccctaaagc

SEQ ID NO: 14359 - RNA, 20 nt, synthetic construct
  source 1..20: mol_type = other RNA
cgctttagggctctggtcct

SEQ ID NO: 14360 - RNA, 20 nt, synthetic construct
  source 1..20: mol_type = other RNA
ccgctttagggctctggtcc

SEQ ID NO: 14361 - RNA, 20 nt, synthetic construct
  source 1..20: mol_type = other RNA
actgtcccgctttagggctc

SEQ ID NO: 14362 - RNA, 20 nt, synthetic construct
  source 1..20: mol_type = other RNA
gagatgactgtcccgcttta

SEQ ID NO: 14363 - RNA, 20 nt, synthetic construct
  source 1..20: mol_type = other RNA
tgagatgactgtcccgcttt

SEQ ID NO: 14364 - RNA, 20 nt, synthetic construct
  source 1..20: mol_type = other RNA
gccctgaagacctcctactc

SEQ ID NO: 14365 - RNA, 20 nt, synthetic construct
  source 1..20: mol_type = other RNA
gcctgagtaggaggtcttca

SEQ ID NO: 14366 - RNA, 20 nt, synthetic construct
  source 1..20: mol_type = other RNA
agcctgagtaggaggtcttc

SEQ ID NO: 14367 - RNA, 20 nt, synthetic construct
  source 1..20: mol_type = other RNA
ggcaggggagcctgagtagg

SEQ ID NO: 14368 - RNA, 20 nt, synthetic construct
  source 1..20: mol_type = other RNA
gggggcaggggagcctgagt

SEQ ID NO: 14369 - RNA, 20 nt, synthetic construct
  source 1..20: mol_type = other RNA
gttagtggtggtgggggcag

SEQ ID NO: 14370 - RNA, 20 nt, synthetic construct
  source 1..20: mol_type = other RNA
tgttagtggtggtgggggca

SEQ ID NO: 14371 - RNA, 20 nt, synthetic construct
  source 1..20: mol_type = other RNA
ttgttagtggtggtgggggc

SEQ ID NO: 14372 - RNA, 20 nt, synthetic construct
  source 1..20: mol_type = other RNA
ttggttgttagtggtggtgg

SEQ ID NO: 14373 - RNA, 20 nt, synthetic construct
  source 1..20: mol_type = other RNA
cttggttgttagtggtggtg

SEQ ID NO: 14374 - RNA, 20 nt, synthetic construct
  source 1..20: mol_type = other RNA
gcttggttgttagtggtggt

SEQ ID NO: 14375 - RNA, 20 nt, synthetic construct
  source 1..20: mol_type = other RNA
tgcttggttgttagtggtgg

SEQ ID NO: 14376 - RNA, 20 nt, synthetic construct
  source 1..20: mol_type = other RNA
agatgcttggttgttagtgg

SEQ ID NO: 14377 - RNA, 20 nt, synthetic construct
  source 1..20: mol_type = other RNA
agaagatgcttggttgttag

SEQ ID NO: 14378 - RNA, 20 nt, synthetic construct
  source 1..20: mol_type = other RNA
ccaagcatcttcttacccgc

SEQ ID NO: 14379 - RNA, 20 nt, synthetic construct
  source 1..20: mol_type = other RNA
ccagcgggtaagaagatgct

SEQ ID NO: 14380 - RNA, 20 nt, synthetic construct
  source 1..20: mol_type = other RNA
cgctggccgcctgcagagac

SEQ ID NO: 14381 - RNA, 20 nt, synthetic construct
  source 1..20: mol_type = other RNA
agtctctgcaggcggccagc

SEQ ID NO: 14382 - RNA, 20 nt, synthetic construct
  source 1..20: mol_type = other RNA
cagtctctgcaggcggccag

SEQ ID NO: 14383 - RNA, 20 nt, synthetic construct
  source 1..20: mol_type = other RNA
tagaagccagtctctgcagg

SEQ ID NO: 14384 - RNA, 20 nt, synthetic construct
  source 1..20: mol_type = other RNA
agagactggcttctacatac

SEQ ID NO: 14385 - RNA, 20 nt, synthetic construct
  source 1..20: mol_type = other RNA
gagactggcttctacatact

SEQ ID NO: 14386 - RNA, 20 nt, synthetic construct
  source 1..20: mol_type = other RNA
tggcttctacatactgggtc

SEQ ID NO: 14387 - RNA, 20 nt, synthetic construct
  source 1..20: mol_type = other RNA
ctacatactgggtcaggttg

SEQ ID NO: 14388 - RNA, 20 nt, synthetic construct
  source 1..20: mol_type = other RNA
tacatactgggtcaggttga

SEQ ID NO: 14389 - RNA, 20 nt, synthetic construct
  source 1..20: mol_type = other RNA
ctgggtcaggttgagggaac

SEQ ID NO: 14390 - RNA, 20 nt, synthetic construct
  source 1..20: mol_type = other RNA
tgggtcaggttgagggaact

SEQ ID NO: 14391 - RNA, 20 nt, synthetic construct
  source 1..20: mol_type = other RNA
cgtagctgctaaagacagag

SEQ ID NO: 14392 - RNA, 20 nt, synthetic construct
  source 1..20: mol_type = other RNA
ctctctgtctttagcagcta

SEQ ID NO: 14393 - RNA, 20 nt, synthetic construct
  source 1..20: mol_type = other RNA
agacagagaggcagcgtcag

SEQ ID NO: 14394 - RNA, 20 nt, synthetic construct
  source 1..20: mol_type = other RNA
aggcagcgtcagtggaactc

SEQ ID NO: 14395 - RNA, 20 nt, synthetic construct
  source 1..20: mol_type = other RNA
ggcagcgtcagtggaactct

SEQ ID NO: 14396 - RNA, 20 nt, synthetic construct
  source 1..20: mol_type = other RNA
aactctgggaccagcactcc

SEQ ID NO: 14397 - RNA, 20 nt, synthetic construct
  source 1..20: mol_type = other RNA
actctgggaccagcactcct

SEQ ID NO: 14398 - RNA, 20 nt, synthetic construct
  source 1..20: mol_type = other RNA
gcactcctgggtccctgtcc

SEQ ID NO: 14399 - RNA, 20 nt, synthetic construct
  source 1..20: mol_type = other RNA
ggacagggacccaggagtgc

SEQ ID NO: 14400 - RNA, 20 nt, synthetic construct
  source 1..20: mol_type = other RNA
gaagaccgggacagggaccc

SEQ ID NO: 14401 - RNA, 20 nt, synthetic construct
  source 1..20: mol_type = other RNA
agagcaggaagaccgggaca

SEQ ID NO: 14402 - RNA, 20 nt, synthetic construct
  source 1..20: mol_type = other RNA
aagagcaggaagaccgggac

SEQ ID NO: 14403 - RNA, 20 nt, synthetic construct
  source 1..20: mol_type = other RNA
aaagaaagagcaggaagacc

SEQ ID NO: 14404 - RNA, 20 nt, synthetic construct
  source 1..20: mol_type = other RNA
caaagaaagagcaggaagac

SEQ ID NO: 14405 - RNA, 20 nt, synthetic construct
  source 1..20: mol_type = other RNA
tgctctttctttgttccatt

SEQ ID NO: 14406 - RNA, 20 nt, synthetic construct
  source 1..20: mol_type = other RNA
gctctttctttgttccattt

SEQ ID NO: 14407 - RNA, 20 nt, synthetic construct
  source 1..20: mol_type = other RNA
aaatggaacaaagaaagagc

SEQ ID NO: 14408 - RNA, 20 nt, synthetic construct
  source 1..20: mol_type = other RNA
attcttgagggaagcccaaa

SEQ ID NO: 14409 - RNA, 20 nt, synthetic construct
  source 1..20: mol_type = other RNA
ttccctcaagaatactccag

SEQ ID NO: 14410 - RNA, 20 nt, synthetic construct
  source 1..20: mol_type = other RNA
cacctctggagtattcttga

SEQ ID NO: 14411 - RNA, 20 nt, synthetic construct
  source 1..20: mol_type = other RNA
gcacctctggagtattcttg

SEQ ID NO: 14412 - RNA, 20 nt, synthetic construct
  source 1..20: mol_type = other RNA
ccagcctggccagcctcggg

SEQ ID NO: 14413 - RNA, 20 nt, synthetic construct
  source 1..20: mol_type = other RNA
cagcctggccagcctcggga

SEQ ID NO: 14414 - RNA, 20 nt, synthetic construct
  source 1..20: mol_type = other RNA
cctcccgaggctggccaggc

SEQ ID NO: 14415 - RNA, 20 nt, synthetic construct
  source 1..20: mol_type = other RNA
atgccctcccgaggctggcc

SEQ ID NO: 14416 - RNA, 20 nt, synthetic construct
  source 1..20: mol_type = other RNA
ggcgaatgccctcccgaggc

SEQ ID NO: 14417 - RNA, 20 nt, synthetic construct
  source 1..20: mol_type = other RNA
cacgggcgaatgccctcccg

SEQ ID NO: 14418 - RNA, 20 nt, synthetic construct
  source 1..20: mol_type = other RNA
ggggcgcggaggagctgcac

SEQ ID NO: 14419 - RNA, 20 nt, synthetic construct
  source 1..20: mol_type = other RNA
gggggcgcggaggagctgca

SEQ ID NO: 14420 - RNA, 20 nt, synthetic construct
  source 1..20: mol_type = other RNA
ggctgggggagggggcgcgg

SEQ ID NO: 14421 - RNA, 20 nt, synthetic construct
  source 1..20: mol_type = other RNA
ggcggctgggggagggggcg

SEQ ID NO: 14422 - RNA, 20 nt, synthetic construct
  source 1..20: mol_type = other RNA
ccctcccccagccgcctcgc

SEQ ID NO: 14423 - RNA, 20 nt, synthetic construct
  source 1..20: mol_type = other RNA
tcccccagccgcctcgccgg

SEQ ID NO: 14424 - RNA, 20 nt, synthetic construct
  source 1..20: mol_type = other RNA
cggcgaggcggctgggggag

SEQ ID NO: 14425 - RNA, 20 nt, synthetic construct
  source 1..20: mol_type = other RNA
ccggcgaggcggctggggga

SEQ ID NO: 14426 - RNA, 20 nt, synthetic construct
  source 1..20: mol_type = other RNA
tccggcgaggcggctggggg

SEQ ID NO: 14427 - RNA, 20 nt, synthetic construct
  source 1..20: mol_type = other RNA
tcctccggcgaggcggctgg

SEQ ID NO: 14428 - RNA, 20 nt, synthetic construct
  source 1..20: mol_type = other RNA
gtcctccggcgaggcggctg

SEQ ID NO: 14429 - RNA, 20 nt, synthetic construct
  source 1..20: mol_type = other RNA
ggtcctccggcgaggcggct

SEQ ID NO: 14430 - RNA, 20 nt, synthetic construct
  source 1..20: mol_type = other RNA
gggtcctccggcgaggcggc

SEQ ID NO: 14431 - RNA, 20 nt, synthetic construct
  source 1..20: mol_type = other RNA
gcctgggtcctccggcgagg

SEQ ID NO: 14432 - RNA, 20 nt, synthetic construct
  source 1..20: mol_type = other RNA
cgccggaggacccaggcgac

SEQ ID NO: 14433 - RNA, 20 nt, synthetic construct
  source 1..20: mol_type = other RNA
gccggaggacccaggcgacg

SEQ ID NO: 14434 - RNA, 20 nt, synthetic construct
  source 1..20: mol_type = other RNA
gtcgcctgggtcctccggcg

SEQ ID NO: 14435 - RNA, 20 nt, synthetic construct
  source 1..20: mol_type = other RNA
ggaggacccaggcgacgggg

SEQ ID NO: 14436 - RNA, 20 nt, synthetic construct
  source 1..20: mol_type = other RNA
gaggacccaggcgacggggc

SEQ ID NO: 14437 - RNA, 20 nt, synthetic construct
  source 1..20: mol_type = other RNA
gccccgtcgcctgggtcctc

SEQ ID NO: 14438 - RNA, 20 nt, synthetic construct
  source 1..20: mol_type = other RNA
gctcgcccgccccgtcgcct

SEQ ID NO: 14439 - RNA, 20 nt, synthetic construct
  source 1..20: mol_type = other RNA
ggctcgcccgccccgtcgcc

SEQ ID NO: 14440 - RNA, 20 nt, synthetic construct
  source 1..20: mol_type = other RNA
gcttccccgcctgactcacc

SEQ ID NO: 14441 - RNA, 20 nt, synthetic construct
  source 1..20: mol_type = other RNA
ggtgagtcaggcggggaagc

SEQ ID NO: 14442 - RNA, 20 nt, synthetic construct
  source 1..20: mol_type = other RNA
cccgcctgactcacctggag

SEQ ID NO: 14443 - RNA, 20 nt, synthetic construct
  source 1..20: mol_type = other RNA
ccgcctgactcacctggagt

SEQ ID NO: 14444 - RNA, 20 nt, synthetic construct
  source 1..20: mol_type = other RNA
cactccaggtgagtcaggcg

SEQ ID NO: 14445 - RNA, 20 nt, synthetic construct
  source 1..20: mol_type = other RNA
ctgactcacctggagtggga

SEQ ID NO: 14446 - RNA, 20 nt, synthetic construct
  source 1..20: mol_type = other RNA
tgactcacctggagtgggag

SEQ ID NO: 14447 - RNA, 20 nt, synthetic construct
  source 1..20: mol_type = other RNA
gactcacctggagtgggagg

SEQ ID NO: 14448 - RNA, 20 nt, synthetic construct
  source 1..20: mol_type = other RNA
cctcccactccaggtgagtc

SEQ ID NO: 14449 - RNA, 20 nt, synthetic construct
  source 1..20: mol_type = other RNA
cacctggagtgggaggggga

SEQ ID NO: 14450 - RNA, 20 nt, synthetic construct
  source 1..20: mol_type = other RNA
acctggagtgggagggggaa

SEQ ID NO: 14451 - RNA, 20 nt, synthetic construct
  source 1..20: mol_type = other RNA
tggagtgggagggggaaggg

SEQ ID NO: 14452 - RNA, 20 nt, synthetic construct
  source 1..20: mol_type = other RNA
tcccttccccctcccactcc

SEQ ID NO: 14453 - RNA, 20 nt, synthetic construct
  source 1..20: mol_type = other RNA
gggagggggaagggaggcgg

SEQ ID NO: 14454 - RNA, 20 nt, synthetic construct
  source 1..20: mol_type = other RNA
agggaggcggcggagccccg

SEQ ID NO: 14455 - RNA, 20 nt, synthetic construct
  source 1..20: mol_type = other RNA
gcggcggagccccgaggtcc

SEQ ID NO: 14456 - RNA, 20 nt, synthetic construct
  source 1..20: mol_type = other RNA
gagccccgaggtcccggcgt

SEQ ID NO: 14457 - RNA, 20 nt, synthetic construct
  source 1..20: mol_type = other RNA
agccccgaggtcccggcgtc

SEQ ID NO: 14458 - RNA, 20 nt, synthetic construct
  source 1..20: mol_type = other RNA
tgcccgacgccgggacctcg

SEQ ID NO: 14459 - RNA, 20 nt, synthetic construct
  source 1..20: mol_type = other RNA
ctgcccgacgccgggacctc

SEQ ID NO: 14460 - RNA, 20 nt, synthetic construct
  source 1..20: mol_type = other RNA
actgcccgacgccgggacct

SEQ ID NO: 14461 - RNA, 20 nt, synthetic construct
  source 1..20: mol_type = other RNA
cccggcgtcgggcagtctct

SEQ ID NO: 14462 - RNA, 20 nt, synthetic construct
  source 1..20: mol_type = other RNA
gcgtcgggcagtctcttgga

SEQ ID NO: 14463 - RNA, 20 nt, synthetic construct
  source 1..20: mol_type = other RNA
ccaagagactgcccgacgcc

SEQ ID NO: 14464 - RNA, 20 nt, synthetic construct
  source 1..20: mol_type = other RNA
tccaagagactgcccgacgc

SEQ ID NO: 14465 - RNA, 20 nt, synthetic construct
  source 1..20: mol_type = other RNA
ggatggagcgtcgcaatgtc

SEQ ID NO: 14466 - RNA, 20 nt, synthetic construct
  source 1..20: mol_type = other RNA
gatggagcgtcgcaatgtcc

SEQ ID NO: 14467 - RNA, 20 nt, synthetic construct
  source 1..20: mol_type = other RNA
atggagcgtcgcaatgtccg

SEQ ID NO: 14468 - RNA, 20 nt, synthetic construct
  source 1..20: mol_type = other RNA
atgtccggggctcgccgtac

SEQ ID NO: 14469 - RNA, 20 nt, synthetic construct
  source 1..20: mol_type = other RNA
tgtccggggctcgccgtact

SEQ ID NO: 14470 - RNA, 20 nt, synthetic construct
  source 1..20: mol_type = other RNA
gtccggggctcgccgtactg

SEQ ID NO: 14471 - RNA, 20 nt, synthetic construct
  source 1..20: mol_type = other RNA
tccggggctcgccgtactgg

SEQ ID NO: 14472 - RNA, 20 nt, synthetic construct
  source 1..20: mol_type = other RNA
ccggggctcgccgtactggg

SEQ ID NO: 14473 - RNA, 20 nt, synthetic construct
  source 1..20: mol_type = other RNA
ccccccagtacggcgagccc

SEQ ID NO: 14474 - RNA, 20 nt, synthetic construct
  source 1..20: mol_type = other RNA
tcgccgtactggggggctcc

SEQ ID NO: 14475 - RNA, 20 nt, synthetic construct
  source 1..20: mol_type = other RNA
cgccgtactggggggctcct

SEQ ID NO: 14476 - RNA, 20 nt, synthetic construct
  source 1..20: mol_type = other RNA
gccgtactggggggctcctg

SEQ ID NO: 14477 - RNA, 20 nt, synthetic construct
  source 1..20: mol_type = other RNA
ccgtactggggggctcctgg

SEQ ID NO: 14478 - RNA, 20 nt, synthetic construct
  source 1..20: mol_type = other RNA
cgtactggggggctcctggg

SEQ ID NO: 14479 - RNA, 20 nt, synthetic construct
  source 1..20: mol_type = other RNA
gtactggggggctcctgggg

SEQ ID NO: 14480 - RNA, 20 nt, synthetic construct
  source 1..20: mol_type = other RNA
cccccaggagccccccagta

SEQ ID NO: 14481 - RNA, 20 nt, synthetic construct
  source 1..20: mol_type = other RNA
ggggggctcctgggggggca

SEQ ID NO: 14482 - RNA, 20 nt, synthetic construct
  source 1..20: mol_type = other RNA
tcctgggggggcacggctct

SEQ ID NO: 14483 - RNA, 20 nt, synthetic construct
  source 1..20: mol_type = other RNA
gggggggcacggctctaggc

SEQ ID NO: 14484 - RNA, 20 nt, synthetic construct
  source 1..20: mol_type = other RNA
ggggggcacggctctaggct

SEQ ID NO: 14485 - RNA, 20 nt, synthetic construct
  source 1..20: mol_type = other RNA
gcctagagccgtgccccccc

SEQ ID NO: 14486 - RNA, 20 nt, synthetic construct
  source 1..20: mol_type = other RNA
gctctaggctgggactgtcc

SEQ ID NO: 14487 - RNA, 20 nt, synthetic construct
  source 1..20: mol_type = other RNA
ctctaggctgggactgtccc

SEQ ID NO: 14488 - RNA, 20 nt, synthetic construct
  source 1..20: mol_type = other RNA
tctaggctgggactgtcccg

SEQ ID NO: 14489 - RNA, 20 nt, synthetic construct
  source 1..20: mol_type = other RNA
gggactgtcccggggcctct

SEQ ID NO: 14490 - RNA, 20 nt, synthetic construct
  source 1..20: mol_type = other RNA
ggcgggctccgagaggcccc

SEQ ID NO: 14491 - RNA, 20 nt, synthetic construct
  source 1..20: mol_type = other RNA
gggcgggctccgagaggccc

SEQ ID NO: 14492 - RNA, 20 nt, synthetic construct
  source 1..20: mol_type = other RNA
gtgggcgggcgggctccgag

SEQ ID NO: 14493 - RNA, 20 nt, synthetic construct
  source 1..20: mol_type = other RNA
gggcggtcacgtgggcgggc

SEQ ID NO: 14494 - RNA, 20 nt, synthetic construct
  source 1..20: mol_type = other RNA
ggggcggtcacgtgggcggg

SEQ ID NO: 14495 - RNA, 20 nt, synthetic construct
  source 1..20: mol_type = other RNA
tttggggcggtcacgtgggc

SEQ ID NO: 14496 - RNA, 20 nt, synthetic construct
  source 1..20: mol_type = other RNA
ttttggggcggtcacgtggg

SEQ ID NO: 14497 - RNA, 20 nt, synthetic construct
  source 1..20: mol_type = other RNA
atattttggggcggtcacgt

SEQ ID NO: 14498 - RNA, 20 nt, synthetic construct
  source 1..20: mol_type = other RNA
gatattttggggcggtcacg

SEQ ID NO: 14499 - RNA, 20 nt, synthetic construct
  source 1..20: mol_type = other RNA
atgtgtcggatattttgggg

SEQ ID NO: 14500 - RNA, 20 nt, synthetic construct
  source 1..20: mol_type = other RNA
aaaatgtgtcggatattttg

SEQ ID NO: 14501 - RNA, 20 nt, synthetic construct
  source 1..20: mol_type = other RNA
gaaaatgtgtcggatatttt

SEQ ID NO: 14502 - RNA, 20 nt, synthetic construct
  source 1..20: mol_type = other RNA
agaaaatgtgtcggatattt

SEQ ID NO: 14503 - RNA, 20 nt, synthetic construct
  source 1..20: mol_type = other RNA
cggtttgggagaaaatgtgt

SEQ ID NO: 14504 - RNA, 20 nt, synthetic construct
  source 1..20: mol_type = other RNA
aaaccgcacactgactctgc

SEQ ID NO: 14505 - RNA, 20 nt, synthetic construct
  source 1..20: mol_type = other RNA
gcagagtcagtgtgcggttt

SEQ ID NO: 14506 - RNA, 20 nt, synthetic construct
  source 1..20: mol_type = other RNA
tgcagagtcagtgtgcggtt

SEQ ID NO: 14507 - RNA, 20 nt, synthetic construct
  source 1..20: mol_type = other RNA
cgcacactgactctgcaggc

SEQ ID NO: 14508 - RNA, 20 nt, synthetic construct
  source 1..20: mol_type = other RNA
gcacactgactctgcaggcg

SEQ ID NO: 14509 - RNA, 20 nt, synthetic construct
  source 1..20: mol_type = other RNA
ccgcctgcagagtcagtgtg

SEQ ID NO: 14510 - RNA, 20 nt, synthetic construct
  source 1..20: mol_type = other RNA
tgactctgcaggcggggaca

SEQ ID NO: 14511 - RNA, 20 nt, synthetic construct
  source 1..20: mol_type = other RNA
ggttggggggggggtgggga

SEQ ID NO: 14512 - RNA, 20 nt, synthetic construct
  source 1..20: mol_type = other RNA
aggttggggggggggtgggg

SEQ ID NO: 14513 - RNA, 20 nt, synthetic construct
  source 1..20: mol_type = other RNA
gggaggttggggggggggtg

SEQ ID NO: 14514 - RNA, 20 nt, synthetic construct
  source 1..20: mol_type = other RNA
agggaggttggggggggggt

SEQ ID NO: 14515 - RNA, 20 nt, synthetic construct
  source 1..20: mol_type = other RNA
gagggaggttgggggggggg

SEQ ID NO: 14516 - RNA, 20 nt, synthetic construct
  source 1..20: mol_type = other RNA
agggagggaggttggggggg

SEQ ID NO: 14517 - RNA, 20 nt, synthetic construct
  source 1..20: mol_type = other RNA
cagggagggaggttgggggg

SEQ ID NO: 14518 - RNA, 20 nt, synthetic construct
  source 1..20: mol_type = other RNA
gcagggagggaggttggggg

SEQ ID NO: 14519 - RNA, 20 nt, synthetic construct
  source 1..20: mol_type = other RNA
ggcagggagggaggttgggg

SEQ ID NO: 14520 - RNA, 20 nt, synthetic construct
  source 1..20: mol_type = other RNA
gggcagggagggaggttggg

SEQ ID NO: 14521 - RNA, 20 nt, synthetic construct
  source 1..20: mol_type = other RNA
tgggcagggagggaggttgg

SEQ ID NO: 14522 - RNA, 20 nt, synthetic construct
  source 1..20: mol_type = other RNA
ttgggcagggagggaggttg

SEQ ID NO: 14523 - RNA, 20 nt, synthetic construct
  source 1..20: mol_type = other RNA
gttgggcagggagggaggtt

SEQ ID NO: 14524 - RNA, 20 nt, synthetic construct
  source 1..20: mol_type = other RNA
agttgggcagggagggaggt

SEQ ID NO: 14525 - RNA, 20 nt, synthetic construct
  source 1..20: mol_type = other RNA
agggagttgggcagggaggg

SEQ ID NO: 14526 - RNA, 20 nt, synthetic construct
  source 1..20: mol_type = other RNA
aggagggagttgggcaggga

SEQ ID NO: 14527 - RNA, 20 nt, synthetic construct
  source 1..20: mol_type = other RNA
gaggagggagttgggcaggg

SEQ ID NO: 14528 - RNA, 20 nt, synthetic construct
  source 1..20: mol_type = other RNA
ggggaggagggagttgggca

SEQ ID NO: 14529 - RNA, 20 nt, synthetic construct
  source 1..20: mol_type = other RNA
gggggaggagggagttgggc

SEQ ID NO: 14530 - RNA, 20 nt, synthetic construct
  source 1..20: mol_type = other RNA
gggagggggaggagggagtt

SEQ ID NO: 14531 - RNA, 20 nt, synthetic construct
  source 1..20: mol_type = other RNA
cgggagggggaggagggagt

SEQ ID NO: 14532 - RNA, 20 nt, synthetic construct
  source 1..20: mol_type = other RNA
cgagggcgggagggggagga

SEQ ID NO: 14533 - RNA, 20 nt, synthetic construct
  source 1..20: mol_type = other RNA
gcgagggcgggagggggagg

SEQ ID NO: 14534 - RNA, 20 nt, synthetic construct
  source 1..20: mol_type = other RNA
ggagcgagggcgggaggggg

SEQ ID NO: 14535 - RNA, 20 nt, synthetic construct
  source 1..20: mol_type = other RNA
ggaggagcgagggcgggagg

SEQ ID NO: 14536 - RNA, 20 nt, synthetic construct
  source 1..20: mol_type = other RNA
gggaggagcgagggcgggag

SEQ ID NO: 14537 - RNA, 20 nt, synthetic construct
  source 1..20: mol_type = other RNA
agggaggagcgagggcggga

SEQ ID NO: 14538 - RNA, 20 nt, synthetic construct
  source 1..20: mol_type = other RNA
gagggaggagcgagggcggg

SEQ ID NO: 14539 - RNA, 20 nt, synthetic construct
  source 1..20: mol_type = other RNA
ggggagggaggagcgagggc

SEQ ID NO: 14540 - RNA, 20 nt, synthetic construct
  source 1..20: mol_type = other RNA
aggggagggaggagcgaggg

SEQ ID NO: 14541 - RNA, 20 nt, synthetic construct
  source 1..20: mol_type = other RNA
ggcaggggagggaggagcga

SEQ ID NO: 14542 - RNA, 20 nt, synthetic construct
  source 1..20: mol_type = other RNA
aggcaggggagggaggagcg

SEQ ID NO: 14543 - RNA, 20 nt, synthetic construct
  source 1..20: mol_type = other RNA
caggggcaggcaggggaggg

SEQ ID NO: 14544 - RNA, 20 nt, synthetic construct
  source 1..20: mol_type = other RNA
gggcaggggcaggcagggga

SEQ ID NO: 14545 - RNA, 20 nt, synthetic construct
  source 1..20: mol_type = other RNA
cgggcaggggcaggcagggg

SEQ ID NO: 14546 - RNA, 20 nt, synthetic construct
  source 1..20: mol_type = other RNA
agccgggcaggggcaggcag

SEQ ID NO: 14547 - RNA, 20 nt, synthetic construct
  source 1..20: mol_type = other RNA
gagccgggcaggggcaggca

SEQ ID NO: 14548 - RNA, 20 nt, synthetic construct
  source 1..20: mol_type = other RNA
ggagccgggcaggggcaggc

SEQ ID NO: 14549 - RNA, 20 nt, synthetic construct
  source 1..20: mol_type = other RNA
ggagggagccgggcaggggc

SEQ ID NO: 14550 - RNA, 20 nt, synthetic construct
  source 1..20: mol_type = other RNA
cagaggagggagccgggcag

SEQ ID NO: 14551 - RNA, 20 nt, synthetic construct
  source 1..20: mol_type = other RNA
acagaggagggagccgggca

SEQ ID NO: 14552 - RNA, 20 nt, synthetic construct
  source 1..20: mol_type = other RNA
cacagaggagggagccgggc

SEQ ID NO: 14553 - RNA, 20 nt, synthetic construct
  source 1..20: mol_type = other RNA
cggctccctcctctgtgccc

SEQ ID NO: 14554 - RNA, 20 nt, synthetic construct
  source 1..20: mol_type = other RNA
ggctccctcctctgtgccct

SEQ ID NO: 14555 - RNA, 20 nt, synthetic construct
  source 1..20: mol_type = other RNA
gctccctcctctgtgccctg

SEQ ID NO: 14556 - RNA, 20 nt, synthetic construct
  source 1..20: mol_type = other RNA
agggcacagaggagggagcc

SEQ ID NO: 14557 - RNA, 20 nt, synthetic construct
  source 1..20: mol_type = other RNA
cagggcacagaggagggagc

SEQ ID NO: 14558 - RNA, 20 nt, synthetic construct
  source 1..20: mol_type = other RNA
cctcctctgtgccctggggc

SEQ ID NO: 14559 - RNA, 20 nt, synthetic construct
  source 1..20: mol_type = other RNA
ctcctctgtgccctggggct

SEQ ID NO: 14560 - RNA, 20 nt, synthetic construct
  source 1..20: mol_type = other RNA
tcctctgtgccctggggctg

SEQ ID NO: 14561 - RNA, 20 nt, synthetic construct
  source 1..20: mol_type = other RNA
cctctgtgccctggggctgg

SEQ ID NO: 14562 - RNA, 20 nt, synthetic construct
  source 1..20: mol_type = other RNA
cagccccagggcacagagga

SEQ ID NO: 14563 - RNA, 20 nt, synthetic construct
  source 1..20: mol_type = other RNA
ccagccccagggcacagagg

SEQ ID NO: 14564 - RNA, 20 nt, synthetic construct
  source 1..20: mol_type = other RNA
tgtgccctggggctgggggg

SEQ ID NO: 14565 - RNA, 20 nt, synthetic construct
  source 1..20: mol_type = other RNA
cccccagccccagggcacag

SEQ ID NO: 14566 - RNA, 20 nt, synthetic construct
  source 1..20: mol_type = other RNA
gccctggggctggggggcgg

SEQ ID NO: 14567 - RNA, 20 nt, synthetic construct
  source 1..20: mol_type = other RNA
ccctggggctggggggcgga

SEQ ID NO: 14568 - RNA, 20 nt, synthetic construct
  source 1..20: mol_type = other RNA
ggggctggggggcggaggga

SEQ ID NO: 14569 - RNA, 20 nt, synthetic construct
  source 1..20: mol_type = other RNA
gggctggggggcggagggat

SEQ ID NO: 14570 - RNA, 20 nt, synthetic construct
  source 1..20: mol_type = other RNA
tccctccgccccccagcccc

SEQ ID NO: 14571 - RNA, 20 nt, synthetic construct
  source 1..20: mol_type = other RNA
ctggggggcggagggatggg

SEQ ID NO: 14572 - RNA, 20 nt, synthetic construct
  source 1..20: mol_type = other RNA
tggggggcggagggatgggt

SEQ ID NO: 14573 - RNA, 20 nt, synthetic construct
  source 1..20: mol_type = other RNA
ggggcggagggatgggtggg

SEQ ID NO: 14574 - RNA, 20 nt, synthetic construct
  source 1..20: mol_type = other RNA
gggcggagggatgggtgggc

SEQ ID NO: 14575 - RNA, 20 nt, synthetic construct
  source 1..20: mol_type = other RNA
cggagggatgggtgggcggg

SEQ ID NO: 14576 - RNA, 20 nt, synthetic construct
  source 1..20: mol_type = other RNA
ggagggatgggtgggcggga

SEQ ID NO: 14577 - RNA, 20 nt, synthetic construct
  source 1..20: mol_type = other RNA
gagggatgggtgggcgggag

SEQ ID NO: 14578 - RNA, 20 nt, synthetic construct
  source 1..20: mol_type = other RNA
agggatgggtgggcgggagg

SEQ ID NO: 14579 - RNA, 20 nt, synthetic construct
  source 1..20: mol_type = other RNA
tgggtgggcgggagggggac

SEQ ID NO: 14580 - RNA, 20 nt, synthetic construct
  source 1..20: mol_type = other RNA
gggtgggcgggagggggact

SEQ ID NO: 14581 - RNA, 20 nt, synthetic construct
  source 1..20: mol_type = other RNA
tgggcgggagggggactggg

SEQ ID NO: 14582 - RNA, 20 nt, synthetic construct
  source 1..20: mol_type = other RNA
gggcgggagggggactgggc

SEQ ID NO: 14583 - RNA, 20 nt, synthetic construct
  source 1..20: mol_type = other RNA
ggcgggagggggactgggcg

SEQ ID NO: 14584 - RNA, 20 nt, synthetic construct
  source 1..20: mol_type = other RNA
gggagggggactgggcgggg

SEQ ID NO: 14585 - RNA, 20 nt, synthetic construct
  source 1..20: mol_type = other RNA
ggggactgggcggggcggcc

SEQ ID NO: 14586 - RNA, 20 nt, synthetic construct
  source 1..20: mol_type = other RNA
gggactgggcggggcggccc

SEQ ID NO: 14587 - RNA, 20 nt, synthetic construct
  source 1..20: mol_type = other RNA
gcggggcggcccgggacgcc

SEQ ID NO: 14588 - RNA, 20 nt, synthetic construct
  source 1..20: mol_type = other RNA
cggggcggcccgggacgcct

SEQ ID NO: 14589 - RNA, 20 nt, synthetic construct
  source 1..20: mol_type = other RNA
ggcagagacccaggcgtccc

SEQ ID NO: 14590 - RNA, 20 nt, synthetic construct
  source 1..20: mol_type = other RNA
gggcagagacccaggcgtcc

SEQ ID NO: 14591 - RNA, 20 nt, synthetic construct
  source 1..20: mol_type = other RNA
aatgggaagggcagagaccc

SEQ ID NO: 14592 - RNA, 20 nt, synthetic construct
  source 1..20: mol_type = other RNA
ctctgcccttcccatttgct

SEQ ID NO: 14593 - RNA, 20 nt, synthetic construct
  source 1..20: mol_type = other RNA
ggaagcctagcaaatgggaa

SEQ ID NO: 14594 - RNA, 20 nt, synthetic construct
  source 1..20: mol_type = other RNA
cggaagcctagcaaatggga

SEQ ID NO: 14595 - RNA, 20 nt, synthetic construct
  source 1..20: mol_type = other RNA
gtcacggaagcctagcaaat

SEQ ID NO: 14596 - RNA, 20 nt, synthetic construct
  source 1..20: mol_type = other RNA
agtcacggaagcctagcaaa

SEQ ID NO: 14597 - RNA, 20 nt, synthetic construct
  source 1..20: mol_type = other RNA
gcttccgtgactccatcctc

SEQ ID NO: 14598 - RNA, 20 nt, synthetic construct
  source 1..20: mol_type = other RNA
cttccgtgactccatcctct

SEQ ID NO: 14599 - RNA, 20 nt, synthetic construct
  source 1..20: mol_type = other RNA
ccgtgactccatcctctggg

SEQ ID NO: 14600 - RNA, 20 nt, synthetic construct
  source 1..20: mol_type = other RNA
gactccatcctctgggaggc

SEQ ID NO: 14601 - RNA, 20 nt, synthetic construct
  source 1..20: mol_type = other RNA
cctcccagaggatggagtca

SEQ ID NO: 14602 - RNA, 20 nt, synthetic construct
  source 1..20: mol_type = other RNA
atcctctgggaggccgggca

SEQ ID NO: 14603 - RNA, 20 nt, synthetic construct
  source 1..20: mol_type = other RNA
gtgcccggcctcccagagga

SEQ ID NO: 14604 - RNA, 20 nt, synthetic construct
  source 1..20: mol_type = other RNA
tctgggaggccgggcacggc

SEQ ID NO: 14605 - RNA, 20 nt, synthetic construct
  source 1..20: mol_type = other RNA
agccgtgcccggcctcccag

SEQ ID NO: 14606 - RNA, 20 nt, synthetic construct
  source 1..20: mol_type = other RNA
aggccgggcacggctggcag

SEQ ID NO: 14607 - RNA, 20 nt, synthetic construct
  source 1..20: mol_type = other RNA
ccgggcacggctggcagagg

SEQ ID NO: 14608 - RNA, 20 nt, synthetic construct
  source 1..20: mol_type = other RNA
cctcctctgccagccgtgcc

SEQ ID NO: 14609 - RNA, 20 nt, synthetic construct
  source 1..20: mol_type = other RNA
ggcagaggaggtcagtgtcc

SEQ ID NO: 14610 - RNA, 20 nt, synthetic construct
  source 1..20: mol_type = other RNA
aaggttggcatcacggggcc

SEQ ID NO: 14611 - RNA, 20 nt, synthetic construct
  source 1..20: mol_type = other RNA
tgatgccaaccttttctctc

SEQ ID NO: 14612 - RNA, 20 nt, synthetic construct
  source 1..20: mol_type = other RNA
agagaaaaggttggcatcac

SEQ ID NO: 14613 - RNA, 20 nt, synthetic construct
  source 1..20: mol_type = other RNA
gagagaaaaggttggcatca

SEQ ID NO: 14614 - RNA, 20 nt, synthetic construct
  source 1..20: mol_type = other RNA
aagtgccagagagaaaaggt

SEQ ID NO: 14615 - RNA, 20 nt, synthetic construct
  source 1..20: mol_type = other RNA
agaaaagtgccagagagaaa

SEQ ID NO: 14616 - RNA, 20 nt, synthetic construct
  source 1..20: mol_type = other RNA
cttttctcctttctgccttt

SEQ ID NO: 14617 - RNA, 20 nt, synthetic construct
  source 1..20: mol_type = other RNA
ttttctcctttctgcctttt

SEQ ID NO: 14618 - RNA, 20 nt, synthetic construct
  source 1..20: mol_type = other RNA
tttctcctttctgccttttg

SEQ ID NO: 14619 - RNA, 20 nt, synthetic construct
  source 1..20: mol_type = other RNA
ttctcctttctgccttttgg

SEQ ID NO: 14620 - RNA, 20 nt, synthetic construct
  source 1..20: mol_type = other RNA
tctcctttctgccttttggg

SEQ ID NO: 14621 - RNA, 20 nt, synthetic construct
  source 1..20: mol_type = other RNA
agtccccccaaaaggcagaa

SEQ ID NO: 14622 - RNA, 20 nt, synthetic construct
  source 1..20: mol_type = other RNA
actcaactagtccccccaaa

SEQ ID NO: 14623 - RNA, 20 nt, synthetic construct
  source 1..20: mol_type = other RNA
gggactagttgagttgtctg

SEQ ID NO: 14624 - RNA, 20 nt, synthetic construct
  source 1..20: mol_type = other RNA
tagttgagttgtctgtggcc

SEQ ID NO: 14625 - RNA, 20 nt, synthetic construct
  source 1..20: mol_type = other RNA
gccaggctgtgactcttgcg

SEQ ID NO: 14626 - RNA, 20 nt, synthetic construct
  source 1..20: mol_type = other RNA
gcctcgcaagagtcacagcc

SEQ ID NO: 14627 - RNA, 20 nt, synthetic construct
  source 1..20: mol_type = other RNA
actcttgcgaggccagtctc

SEQ ID NO: 14628 - RNA, 20 nt, synthetic construct
  source 1..20: mol_type = other RNA
ccagtctctggcgcctcccc

SEQ ID NO: 14629 - RNA, 20 nt, synthetic construct
  source 1..20: mol_type = other RNA
cagtctctggcgcctcccca

SEQ ID NO: 14630 - RNA, 20 nt, synthetic construct
  source 1..20: mol_type = other RNA
cctggggaggcgccagagac

SEQ ID NO: 14631 - RNA, 20 nt, synthetic construct
  source 1..20: mol_type = other RNA
cgcctccccagggtaggcaa

SEQ ID NO: 14632 - RNA, 20 nt, synthetic construct
  source 1..20: mol_type = other RNA
gcctccccagggtaggcaat

SEQ ID NO: 14633 - RNA, 20 nt, synthetic construct
  source 1..20: mol_type = other RNA
cctccccagggtaggcaatg

SEQ ID NO: 14634 - RNA, 20 nt, synthetic construct
  source 1..20: mol_type = other RNA
ccccagggtaggcaatgggg

SEQ ID NO: 14635 - RNA, 20 nt, synthetic construct
  source 1..20: mol_type = other RNA
ccccattgcctaccctgggg

SEQ ID NO: 14636 - RNA, 20 nt, synthetic construct
  source 1..20: mol_type = other RNA
ccgccccattgcctaccctg

SEQ ID NO: 14637 - RNA, 20 nt, synthetic construct
  source 1..20: mol_type = other RNA
accgccccattgcctaccct

SEQ ID NO: 14638 - RNA, 20 nt, synthetic construct
  source 1..20: mol_type = other RNA
taccgccccattgcctaccc

SEQ ID NO: 14639 - RNA, 20 nt, synthetic construct
  source 1..20: mol_type = other RNA
tacccactccctcccagtgc

SEQ ID NO: 14640 - RNA, 20 nt, synthetic construct
  source 1..20: mol_type = other RNA
actccctcccagtgctggat

SEQ ID NO: 14641 - RNA, 20 nt, synthetic construct
  source 1..20: mol_type = other RNA
atccagcactgggagggagt

SEQ ID NO: 14642 - RNA, 20 nt, synthetic construct
  source 1..20: mol_type = other RNA
aatccagcactgggagggag

SEQ ID NO: 14643 - RNA, 20 nt, synthetic construct
  source 1..20: mol_type = other RNA
cctcccagtgctggattggc

SEQ ID NO: 14644 - RNA, 20 nt, synthetic construct
  source 1..20: mol_type = other RNA
ctcccagtgctggattggcc

SEQ ID NO: 14645 - RNA, 20 nt, synthetic construct
  source 1..20: mol_type = other RNA
cggccaatccagcactggga

SEQ ID NO: 14646 - RNA, 20 nt, synthetic construct
  source 1..20: mol_type = other RNA
cagtgctggattggccgggc

SEQ ID NO: 14647 - RNA, 20 nt, synthetic construct
  source 1..20: mol_type = other RNA
tgcccggccaatccagcact

SEQ ID NO: 14648 - RNA, 20 nt, synthetic construct
  source 1..20: mol_type = other RNA
ctgcccggccaatccagcac

SEQ ID NO: 14649 - RNA, 20 nt, synthetic construct
  source 1..20: mol_type = other RNA
agatctggcatactcctgcc

SEQ ID NO: 14650 - RNA, 20 nt, synthetic construct
  source 1..20: mol_type = other RNA
aggagcatctattctagatc

SEQ ID NO: 14651 - RNA, 20 nt, synthetic construct
  source 1..20: mol_type = other RNA
gctgagcaaagagtaagggc

SEQ ID NO: 14652 - RNA, 20 nt, synthetic construct
  source 1..20: mol_type = other RNA
gaaggctgagcaaagagtaa

SEQ ID NO: 14653 - RNA, 20 nt, synthetic construct
  source 1..20: mol_type = other RNA
tgaaggctgagcaaagagta

SEQ ID NO: 14654 - RNA, 20 nt, synthetic construct
  source 1..20: mol_type = other RNA
ctacttggatctgcaggtga

SEQ ID NO: 14655 - RNA, 20 nt, synthetic construct
  source 1..20: mol_type = other RNA
gagaggctacttggatctgc

SEQ ID NO: 14656 - RNA, 20 nt, synthetic construct
  source 1..20: mol_type = other RNA
aggggaagggagaggctact

SEQ ID NO: 14657 - RNA, 20 nt, synthetic construct
  source 1..20: mol_type = other RNA
ggtgggctaggggaagggag

SEQ ID NO: 14658 - RNA, 20 nt, synthetic construct
  source 1..20: mol_type = other RNA
actgaggtgggctaggggaa

SEQ ID NO: 14659 - RNA, 20 nt, synthetic construct
  source 1..20: mol_type = other RNA
gactgaggtgggctagggga

SEQ ID NO: 14660 - RNA, 20 nt, synthetic construct
  source 1..20: mol_type = other RNA
cctagcccacctcagtcctt

SEQ ID NO: 14661 - RNA, 20 nt, synthetic construct
  source 1..20: mol_type = other RNA
aaaggactgaggtgggctag

SEQ ID NO: 14662 - RNA, 20 nt, synthetic construct
  source 1..20: mol_type = other RNA
caaaggactgaggtgggcta

SEQ ID NO: 14663 - RNA, 20 nt, synthetic construct
  source 1..20: mol_type = other RNA
ccaaaggactgaggtgggct

SEQ ID NO: 14664 - RNA, 20 nt, synthetic construct
  source 1..20: mol_type = other RNA
cacctcagtcctttggtccc

SEQ ID NO: 14665 - RNA, 20 nt, synthetic construct
  source 1..20: mol_type = other RNA
tgggaccaaaggactgaggt

SEQ ID NO: 14666 - RNA, 20 nt, synthetic construct
  source 1..20: mol_type = other RNA
ctgggaccaaaggactgagg

SEQ ID NO: 14667 - RNA, 20 nt, synthetic construct
  source 1..20: mol_type = other RNA
ctcctgggaccaaaggactg

SEQ ID NO: 14668 - RNA, 20 nt, synthetic construct
  source 1..20: mol_type = other RNA
ctttggtcccaggagcaaac

SEQ ID NO: 14669 - RNA, 20 nt, synthetic construct
  source 1..20: mol_type = other RNA
cagtttgctcctgggaccaa

SEQ ID NO: 14670 - RNA, 20 nt, synthetic construct
  source 1..20: mol_type = other RNA
ggagcaaactggttgactag

SEQ ID NO: 14671 - RNA, 20 nt, synthetic construct
  source 1..20: mol_type = other RNA
tagtcaaccagtttgctcct

SEQ ID NO: 14672 - RNA, 20 nt, synthetic construct
  source 1..20: mol_type = other RNA
ctagtcaaccagtttgctcc

SEQ ID NO: 14673 - RNA, 20 nt, synthetic construct
  source 1..20: mol_type = other RNA
ggttgactagtggctgttgc

SEQ ID NO: 14674 - RNA, 20 nt, synthetic construct
  source 1..20: mol_type = other RNA
gttgactagtggctgttgct

SEQ ID NO: 14675 - RNA, 20 nt, synthetic construct
  source 1..20: mol_type = other RNA
ttgactagtggctgttgctg

SEQ ID NO: 14676 - RNA, 20 nt, synthetic construct
  source 1..20: mol_type = other RNA
tgactagtggctgttgctgg

SEQ ID NO: 14677 - RNA, 20 nt, synthetic construct
  source 1..20: mol_type = other RNA
ggctgttgctgggggtgctg

SEQ ID NO: 14678 - RNA, 20 nt, synthetic construct
  source 1..20: mol_type = other RNA
ttgctgggggtgctgaggcc

SEQ ID NO: 14679 - RNA, 20 nt, synthetic construct
  source 1..20: mol_type = other RNA
tgctgggggtgctgaggcca

SEQ ID NO: 14680 - RNA, 20 nt, synthetic construct
  source 1..20: mol_type = other RNA
gggaagatgtctgtgagccc

SEQ ID NO: 14681 - RNA, 20 nt, synthetic construct
  source 1..20: mol_type = other RNA
atcttccctgtcatcttgcc

SEQ ID NO: 14682 - RNA, 20 nt, synthetic construct
  source 1..20: mol_type = other RNA
ttactccaggcaagatgaca

SEQ ID NO: 14683 - RNA, 20 nt, synthetic construct
  source 1..20: mol_type = other RNA
cttactccaggcaagatgac

SEQ ID NO: 14684 - RNA, 20 nt, synthetic construct
  source 1..20: mol_type = other RNA
tcttgcctggagtaagctcc

SEQ ID NO: 14685 - RNA, 20 nt, synthetic construct
  source 1..20: mol_type = other RNA
tggagtaagctccaggagtt

SEQ ID NO: 14686 - RNA, 20 nt, synthetic construct
  source 1..20: mol_type = other RNA
ggagtaagctccaggagtta

SEQ ID NO: 14687 - RNA, 20 nt, synthetic construct
  source 1..20: mol_type = other RNA
taactcctggagcttactcc

SEQ ID NO: 14688 - RNA, 20 nt, synthetic construct
  source 1..20: mol_type = other RNA
gctccaggagttagggcgcc

SEQ ID NO: 14689 - RNA, 20 nt, synthetic construct
  source 1..20: mol_type = other RNA
ctccaggagttagggcgcct

SEQ ID NO: 14690 - RNA, 20 nt, synthetic construct
  source 1..20: mol_type = other RNA
gacccaggcgccctaactcc

SEQ ID NO: 14691 - RNA, 20 nt, synthetic construct
  source 1..20: mol_type = other RNA
caactggcagccagggaccc

SEQ ID NO: 14692 - RNA, 20 nt, synthetic construct
  source 1..20: mol_type = other RNA
tgggggacaactggcagcca

SEQ ID NO: 14693 - RNA, 20 nt, synthetic construct
  source 1..20: mol_type = other RNA
gtgggggacaactggcagcc

SEQ ID NO: 14694 - RNA, 20 nt, synthetic construct
  source 1..20: mol_type = other RNA
gccagttgtcccccaccttt

SEQ ID NO: 14695 - RNA, 20 nt, synthetic construct
  source 1..20: mol_type = other RNA
ttgtcccccacctttaggcc

SEQ ID NO: 14696 - RNA, 20 nt, synthetic construct
  source 1..20: mol_type = other RNA
gcctaaaggtgggggacaac

SEQ ID NO: 14697 - RNA, 20 nt, synthetic construct
  source 1..20: mol_type = other RNA
cccacctttaggcctggatt

SEQ ID NO: 14698 - RNA, 20 nt, synthetic construct
  source 1..20: mol_type = other RNA
aaatccaggcctaaaggtgg

SEQ ID NO: 14699 - RNA, 20 nt, synthetic construct
  source 1..20: mol_type = other RNA
cctttaggcctggatttgga

SEQ ID NO: 14700 - RNA, 20 nt, synthetic construct
  source 1..20: mol_type = other RNA
ctttaggcctggatttggaa

SEQ ID NO: 14701 - RNA, 20 nt, synthetic construct
  source 1..20: mol_type = other RNA
tccaaatccaggcctaaagg

SEQ ID NO: 14702 - RNA, 20 nt, synthetic construct
  source 1..20: mol_type = other RNA
ccttccaaatccaggcctaa

SEQ ID NO: 14703 - RNA, 20 nt, synthetic construct
  source 1..20: mol_type = other RNA
gcctggatttggaaggggag

SEQ ID NO: 14704 - RNA, 20 nt, synthetic construct
  source 1..20: mol_type = other RNA
ggatttggaaggggagaggc

SEQ ID NO: 14705 - RNA, 20 nt, synthetic construct
  source 1..20: mol_type = other RNA
gcctctccccttccaaatcc

SEQ ID NO: 14706 - RNA, 20 nt, synthetic construct
  source 1..20: mol_type = other RNA
tggaaggggagaggctggag

SEQ ID NO: 14707 - RNA, 20 nt, synthetic construct
  source 1..20: mol_type = other RNA
aaggggagaggctggagagg

SEQ ID NO: 14708 - RNA, 20 nt, synthetic construct
  source 1..20: mol_type = other RNA
aggggagaggctggagagga

SEQ ID NO: 14709 - RNA, 20 nt, synthetic construct
  source 1..20: mol_type = other RNA
gagaggctggagaggagggc

SEQ ID NO: 14710 - RNA, 20 nt, synthetic construct
  source 1..20: mol_type = other RNA
aggctggagaggagggcagg

SEQ ID NO: 14711 - RNA, 20 nt, synthetic construct
  source 1..20: mol_type = other RNA
gaggagggcaggaggaactg

SEQ ID NO: 14712 - RNA, 20 nt, synthetic construct
  source 1..20: mol_type = other RNA
agggcaggaggaactgtggc

SEQ ID NO: 14713 - RNA, 20 nt, synthetic construct
  source 1..20: mol_type = other RNA
gggcaggaggaactgtggct

SEQ ID NO: 14714 - RNA, 20 nt, synthetic construct
  source 1..20: mol_type = other RNA
ggaggaactgtggctgggag

SEQ ID NO: 14715 - RNA, 20 nt, synthetic construct
  source 1..20: mol_type = other RNA
gaggaactgtggctgggagt

SEQ ID NO: 14716 - RNA, 20 nt, synthetic construct
  source 1..20: mol_type = other RNA
gaactgtggctgggagtggg

SEQ ID NO: 14717 - RNA, 20 nt, synthetic construct
  source 1..20: mol_type = other RNA
gctgggagtgggaggagcct

SEQ ID NO: 14718 - RNA, 20 nt, synthetic construct
  source 1..20: mol_type = other RNA
ctgggagtgggaggagcctt

SEQ ID NO: 14719 - RNA, 20 nt, synthetic construct
  source 1..20: mol_type = other RNA
gagtgggaggagccttgggc

SEQ ID NO: 14720 - RNA, 20 nt, synthetic construct
  source 1..20: mol_type = other RNA
agtgggaggagccttgggct

SEQ ID NO: 14721 - RNA, 20 nt, synthetic construct
  source 1..20: mol_type = other RNA
tctctctcacacccagccca

SEQ ID NO: 14722 - RNA, 20 nt, synthetic construct
  source 1..20: mol_type = other RNA
gggtgtgagagagaaagccc

SEQ ID NO: 14723 - RNA, 20 nt, synthetic construct
  source 1..20: mol_type = other RNA
gagagagaaagcccaggcag

SEQ ID NO: 14724 - RNA, 20 nt, synthetic construct
  source 1..20: mol_type = other RNA
agagagaaagcccaggcaga

SEQ ID NO: 14725 - RNA, 20 nt, synthetic construct
  source 1..20: mol_type = other RNA
cagacacacaccctctgcct

SEQ ID NO: 14726 - RNA, 20 nt, synthetic construct
  source 1..20: mol_type = other RNA
gcagacacacaccctctgcc

SEQ ID NO: 14727 - RNA, 20 nt, synthetic construct
  source 1..20: mol_type = other RNA
gtgtctgccctagccagcac

SEQ ID NO: 14728 - RNA, 20 nt, synthetic construct
  source 1..20: mol_type = other RNA
aggcaggccggtgctggcta

SEQ ID NO: 14729 - RNA, 20 nt, synthetic construct
  source 1..20: mol_type = other RNA
caggcaggccggtgctggct

SEQ ID NO: 14730 - RNA, 20 nt, synthetic construct
  source 1..20: mol_type = other RNA
gcaggcaggcaggccggtgc

SEQ ID NO: 14731 - RNA, 20 nt, synthetic construct
  source 1..20: mol_type = other RNA
ggcctgcctgcctgcctgcc

SEQ ID NO: 14732 - RNA, 20 nt, synthetic construct
  source 1..20: mol_type = other RNA
aggcaggcaggcaggcaggc

SEQ ID NO: 14733 - RNA, 20 nt, synthetic construct
  source 1..20: mol_type = other RNA
taccaggcaggcaggcaggc

SEQ ID NO: 14734 - RNA, 20 nt, synthetic construct
  source 1..20: mol_type = other RNA
catctaccaggcaggcaggc

SEQ ID NO: 14735 - RNA, 20 nt, synthetic construct
  source 1..20: mol_type = other RNA
ggcacatctaccaggcaggc

SEQ ID NO: 14736 - RNA, 20 nt, synthetic construct
  source 1..20: mol_type = other RNA
tcatggcacatctaccaggc

SEQ ID NO: 14737 - RNA, 20 nt, synthetic construct
  source 1..20: mol_type = other RNA
gcattcatggcacatctacc

SEQ ID NO: 14738 - RNA, 20 nt, synthetic construct
  source 1..20: mol_type = other RNA
gccatgaatgctgttgactc

SEQ ID NO: 14739 - RNA, 20 nt, synthetic construct
  source 1..20: mol_type = other RNA
ccatgaatgctgttgactcc

SEQ ID NO: 14740 - RNA, 20 nt, synthetic construct
  source 1..20: mol_type = other RNA
cccggagtcaacagcattca

SEQ ID NO: 14741 - RNA, 20 nt, synthetic construct
  source 1..20: mol_type = other RNA
cacgcacacacacacacacc

SEQ ID NO: 14742 - RNA, 20 nt, synthetic construct
  source 1..20: mol_type = other RNA
cagacactcactctcggcac

SEQ ID NO: 14743 - RNA, 20 nt, synthetic construct
  source 1..20: mol_type = other RNA
gagtgagtgtctgtgtctga

SEQ ID NO: 14744 - RNA, 20 nt, synthetic construct
  source 1..20: mol_type = other RNA
agtgagtgtctgtgtctgat

SEQ ID NO: 14745 - RNA, 20 nt, synthetic construct
  source 1..20: mol_type = other RNA
gtgagtgtctgtgtctgatg

SEQ ID NO: 14746 - RNA, 20 nt, synthetic construct
  source 1..20: mol_type = other RNA
tgagtgtctgtgtctgatgg

SEQ ID NO: 14747 - RNA, 20 nt, synthetic construct
  source 1..20: mol_type = other RNA
cctagagtgagagaacccag

SEQ ID NO: 14748 - RNA, 20 nt, synthetic construct
  source 1..20: mol_type = other RNA
cactgggttctctcactcta

SEQ ID NO: 14749 - RNA, 20 nt, synthetic construct
  source 1..20: mol_type = other RNA
ccactgggttctctcactct

SEQ ID NO: 14750 - RNA, 20 nt, synthetic construct
  source 1..20: mol_type = other RNA
gaatgcagagtgaaaccact

SEQ ID NO: 14751 - RNA, 20 nt, synthetic construct
  source 1..20: mol_type = other RNA
agaatgcagagtgaaaccac

SEQ ID NO: 14752 - RNA, 20 nt, synthetic construct
  source 1..20: mol_type = other RNA
tttcactctgcattctactg

SEQ ID NO: 14753 - RNA, 20 nt, synthetic construct
  source 1..20: mol_type = other RNA
ctgcattctactgaggacag

SEQ ID NO: 14754 - RNA, 20 nt, synthetic construct
  source 1..20: mol_type = other RNA
tgcattctactgaggacaga

SEQ ID NO: 14755 - RNA, 20 nt, synthetic construct
  source 1..20: mol_type = other RNA
gacagagggagagaaaagaa

SEQ ID NO: 14756 - RNA, 20 nt, synthetic construct
  source 1..20: mol_type = other RNA
acagagggagagaaaagaat

SEQ ID NO: 14757 - RNA, 20 nt, synthetic construct
  source 1..20: mol_type = other RNA
tgcagtccaagctctgtgca

SEQ ID NO: 14758 - RNA, 20 nt, synthetic construct
  source 1..20: mol_type = other RNA
tgggatccgtgcacagagct

SEQ ID NO: 14759 - RNA, 20 nt, synthetic construct
  source 1..20: mol_type = other RNA
acggatcccaaacactccca

SEQ ID NO: 14760 - RNA, 20 nt, synthetic construct
  source 1..20: mol_type = other RNA
cggatcccaaacactcccat

SEQ ID NO: 14761 - RNA, 20 nt, synthetic construct
  source 1..20: mol_type = other RNA
ggatcccaaacactcccatg

SEQ ID NO: 14762 - RNA, 20 nt, synthetic construct
  source 1..20: mol_type = other RNA
ccaaacactcccatggggac

SEQ ID NO: 14763 - RNA, 20 nt, synthetic construct
  source 1..20: mol_type = other RNA
cagtccccatgggagtgttt

SEQ ID NO: 14764 - RNA, 20 nt, synthetic construct
  source 1..20: mol_type = other RNA
ccagtccccatgggagtgtt

SEQ ID NO: 14765 - RNA, 20 nt, synthetic construct
  source 1..20: mol_type = other RNA
actcccatggggactggagt

SEQ ID NO: 14766 - RNA, 20 nt, synthetic construct
  source 1..20: mol_type = other RNA
ctcccatggggactggagtt

SEQ ID NO: 14767 - RNA, 20 nt, synthetic construct
  source 1..20: mol_type = other RNA
ccatggggactggagttggg

SEQ ID NO: 14768 - RNA, 20 nt, synthetic construct
  source 1..20: mol_type = other RNA
catggggactggagttggga

SEQ ID NO: 14769 - RNA, 20 nt, synthetic construct
  source 1..20: mol_type = other RNA
ctcccaactccagtccccat

SEQ ID NO: 14770 - RNA, 20 nt, synthetic construct
  source 1..20: mol_type = other RNA
cctcccaactccagtcccca

SEQ ID NO: 14771 - RNA, 20 nt, synthetic construct
  source 1..20: mol_type = other RNA
tggagttgggagggagaaag

SEQ ID NO: 14772 - RNA, 20 nt, synthetic construct
  source 1..20: mol_type = other RNA
tgggagggagaaagaggaga

SEQ ID NO: 14773 - RNA, 20 nt, synthetic construct
  source 1..20: mol_type = other RNA
gggagggagaaagaggagaa

SEQ ID NO: 14774 - RNA, 20 nt, synthetic construct
  source 1..20: mol_type = other RNA
ggagggagaaagaggagaag

SEQ ID NO: 14775 - RNA, 20 nt, synthetic construct
  source 1..20: mol_type = other RNA
agaaggggagagtctgagct

SEQ ID NO: 14776 - RNA, 20 nt, synthetic construct
  source 1..20: mol_type = other RNA
agagtctgagctaggctgat

SEQ ID NO: 14777 - RNA, 20 nt, synthetic construct
  source 1..20: mol_type = other RNA
tctgagctaggctgataggc

SEQ ID NO: 14778 - RNA, 20 nt, synthetic construct
  source 1..20: mol_type = other RNA
attgctggggaaggtacttt

SEQ ID NO: 14779 - RNA, 20 nt, synthetic construct
  source 1..20: mol_type = other RNA
cattgctggggaaggtactt

SEQ ID NO: 14780 - RNA, 20 nt, synthetic construct
  source 1..20: mol_type = other RNA
ccttccccagcaatgctcgc

SEQ ID NO: 14781 - RNA, 20 nt, synthetic construct
  source 1..20: mol_type = other RNA
cttccccagcaatgctcgca

SEQ ID NO: 14782 - RNA, 20 nt, synthetic construct
  source 1..20: mol_type = other RNA
cctgcgagcattgctgggga

SEQ ID NO: 14783 - RNA, 20 nt, synthetic construct
  source 1..20: mol_type = other RNA
gcaatgctcgcagggtgacc

SEQ ID NO: 14784 - RNA, 20 nt, synthetic construct
  source 1..20: mol_type = other RNA
gtcaccctgcgagcattgct

SEQ ID NO: 14785 - RNA, 20 nt, synthetic construct
  source 1..20: mol_type = other RNA
ggtcaccctgcgagcattgc

SEQ ID NO: 14786 - RNA, 20 nt, synthetic construct
  source 1..20: mol_type = other RNA
ctcgcagggtgaccaggacc

SEQ ID NO: 14787 - RNA, 20 nt, synthetic construct
  source 1..20: mol_type = other RNA
tcgcagggtgaccaggacct

SEQ ID NO: 14788 - RNA, 20 nt, synthetic construct
  source 1..20: mol_type = other RNA
ggacctgggacacagactcc

SEQ ID NO: 14789 - RNA, 20 nt, synthetic construct
  source 1..20: mol_type = other RNA
gacctgggacacagactcct

SEQ ID NO: 14790 - RNA, 20 nt, synthetic construct
  source 1..20: mol_type = other RNA
ggagtctgtgtcccaggtcc

SEQ ID NO: 14791 - RNA, 20 nt, synthetic construct
  source 1..20: mol_type = other RNA
gacccaggagtctgtgtccc

SEQ ID NO: 14792 - RNA, 20 nt, synthetic construct
  source 1..20: mol_type = other RNA
tggaaaatgtgacgtgaccc

SEQ ID NO: 14793 - RNA, 20 nt, synthetic construct
  source 1..20: mol_type = other RNA
tcacgtcacattttccatac

SEQ ID NO: 14794 - RNA, 20 nt, synthetic construct
  source 1..20: mol_type = other RNA
ttttccatactggaattact

SEQ ID NO: 14795 - RNA, 20 nt, synthetic construct
  source 1..20: mol_type = other RNA
aaagccaagtaattccagta

SEQ ID NO: 14796 - RNA, 20 nt, synthetic construct
  source 1..20: mol_type = other RNA
gctttgtccttgctcccccc

SEQ ID NO: 14797 - RNA, 20 nt, synthetic construct
  source 1..20: mol_type = other RNA
ctttgtccttgctcccccct

SEQ ID NO: 14798 - RNA, 20 nt, synthetic construct
  source 1..20: mol_type = other RNA
tttgtccttgctcccccctg

SEQ ID NO: 14799 - RNA, 20 nt, synthetic construct
  source 1..20: mol_type = other RNA
ttgtccttgctcccccctgg

SEQ ID NO: 14800 - RNA, 20 nt, synthetic construct
  source 1..20: mol_type = other RNA
cttgctcccccctgggggcc

SEQ ID NO: 14801 - RNA, 20 nt, synthetic construct
  source 1..20: mol_type = other RNA
ctggcccccaggggggagca

SEQ ID NO: 14802 - RNA, 20 nt, synthetic construct
  source 1..20: mol_type = other RNA
aggacacctggcccccaggg

SEQ ID NO: 14803 - RNA, 20 nt, synthetic construct
  source 1..20: mol_type = other RNA
gaggacacctggcccccagg

SEQ ID NO: 14804 - RNA, 20 nt, synthetic construct
  source 1..20: mol_type = other RNA
ggaggacacctggcccccag

SEQ ID NO: 14805 - RNA, 20 nt, synthetic construct
  source 1..20: mol_type = other RNA
gggaggacacctggccccca

SEQ ID NO: 14806 - RNA, 20 nt, synthetic construct
  source 1..20: mol_type = other RNA
agggaggacacctggccccc

SEQ ID NO: 14807 - RNA, 20 nt, synthetic construct
  source 1..20: mol_type = other RNA
ggccaggtgtcctccctcct

SEQ ID NO: 14808 - RNA, 20 nt, synthetic construct
  source 1..20: mol_type = other RNA
ggtgtcctccctcctgggaa

SEQ ID NO: 14809 - RNA, 20 nt, synthetic construct
  source 1..20: mol_type = other RNA
ttcccaggagggaggacacc

SEQ ID NO: 14810 - RNA, 20 nt, synthetic construct
  source 1..20: mol_type = other RNA
agcagcctttcccaggaggg

SEQ ID NO: 14811 - RNA, 20 nt, synthetic construct
  source 1..20: mol_type = other RNA
aaaagcagcctttcccagga

SEQ ID NO: 14812 - RNA, 20 nt, synthetic construct
  source 1..20: mol_type = other RNA
caaaagcagcctttcccagg

SEQ ID NO: 14813 - RNA, 20 nt, synthetic construct
  source 1..20: mol_type = other RNA
taccaaaagcagcctttccc

SEQ ID NO: 14814 - RNA, 20 nt, synthetic construct
  source 1..20: mol_type = other RNA
tgcttttggtagccaaagtc

SEQ ID NO: 14815 - RNA, 20 nt, synthetic construct
  source 1..20: mol_type = other RNA
tggtagccaaagtcaggtga

SEQ ID NO: 14816 - RNA, 20 nt, synthetic construct
  source 1..20: mol_type = other RNA
ccaaagtcaggtgaaggaga

SEQ ID NO: 14817 - RNA, 20 nt, synthetic construct
  source 1..20: mol_type = other RNA
caaagtcaggtgaaggagat

SEQ ID NO: 14818 - RNA, 20 nt, synthetic construct
  source 1..20: mol_type = other RNA
aaagtcaggtgaaggagatg

SEQ ID NO: 14819 - RNA, 20 nt, synthetic construct
  source 1..20: mol_type = other RNA
aagtcaggtgaaggagatgg

SEQ ID NO: 14820 - RNA, 20 nt, synthetic construct
  source 1..20: mol_type = other RNA
ccatctccttcacctgactt

SEQ ID NO: 14821 - RNA, 20 nt, synthetic construct
  source 1..20: mol_type = other RNA
aaggagatgggggaaagaag

SEQ ID NO: 14822 - RNA, 20 nt, synthetic construct
  source 1..20: mol_type = other RNA
gggaaagaagaggcatgctg

SEQ ID NO: 14823 - RNA, 20 nt, synthetic construct
  source 1..20: mol_type = other RNA
aggcatgctgtggttacctc

SEQ ID NO: 14824 - RNA, 20 nt, synthetic construct
  source 1..20: mol_type = other RNA
ggcatgctgtggttacctca

SEQ ID NO: 14825 - RNA, 20 nt, synthetic construct
  source 1..20: mol_type = other RNA
gctgtggttacctcagggaa

SEQ ID NO: 14826 - RNA, 20 nt, synthetic construct
  source 1..20: mol_type = other RNA
ctgtggttacctcagggaat

SEQ ID NO: 14827 - RNA, 20 nt, synthetic construct
  source 1..20: mol_type = other RNA
ttacctcagggaatgggaga

SEQ ID NO: 14828 - RNA, 20 nt, synthetic construct
  source 1..20: mol_type = other RNA
cagggaatgggagatggcaa

SEQ ID NO: 14829 - RNA, 20 nt, synthetic construct
  source 1..20: mol_type = other RNA
agggaatgggagatggcaat

SEQ ID NO: 14830 - RNA, 20 nt, synthetic construct
  source 1..20: mol_type = other RNA
ttgccatctcccattccctg

SEQ ID NO: 14831 - RNA, 20 nt, synthetic construct
  source 1..20: mol_type = other RNA
ggaatgggagatggcaatgg

SEQ ID NO: 14832 - RNA, 20 nt, synthetic construct
  source 1..20: mol_type = other RNA
caagccctctctttcactcc

SEQ ID NO: 14833 - RNA, 20 nt, synthetic construct
  source 1..20: mol_type = other RNA
aagccctctctttcactcca

SEQ ID NO: 14834 - RNA, 20 nt, synthetic construct
  source 1..20: mol_type = other RNA
ctctctttcactccagggat

SEQ ID NO: 14835 - RNA, 20 nt, synthetic construct
  source 1..20: mol_type = other RNA
tatccctggagtgaaagaga

SEQ ID NO: 14836 - RNA, 20 nt, synthetic construct
  source 1..20: mol_type = other RNA
ctatccctggagtgaaagag

SEQ ID NO: 14837 - RNA, 20 nt, synthetic construct
  source 1..20: mol_type = other RNA
ctccagggataggaagagct

SEQ ID NO: 14838 - RNA, 20 nt, synthetic construct
  source 1..20: mol_type = other RNA
ttcctagctcttcctatccc

SEQ ID NO: 14839 - RNA, 20 nt, synthetic construct
  source 1..20: mol_type = other RNA
gccacctggggacgggaccc

SEQ ID NO: 14840 - RNA, 20 nt, synthetic construct
  source 1..20: mol_type = other RNA
ccttactggtgggaaccaaa

SEQ ID NO: 14841 - RNA, 20 nt, synthetic construct
  source 1..20: mol_type = other RNA
gagatctcgtcagggccttt

SEQ ID NO: 14842 - RNA, 20 nt, synthetic construct
  source 1..20: mol_type = other RNA
gccctgacgagatctccaac

SEQ ID NO: 14843 - RNA, 20 nt, synthetic construct
  source 1..20: mol_type = other RNA
gcctgttggagatctcgtca

SEQ ID NO: 14844 - RNA, 20 nt, synthetic construct
  source 1..20: mol_type = other RNA
agcctgttggagatctcgtc

SEQ ID NO: 14845 - RNA, 20 nt, synthetic construct
  source 1..20: mol_type = other RNA
atctccaacaggctatacaa

SEQ ID NO: 14846 - RNA, 20 nt, synthetic construct
  source 1..20: mol_type = other RNA
tctccaacaggctatacaat

SEQ ID NO: 14847 - RNA, 20 nt, synthetic construct
  source 1..20: mol_type = other RNA
aggcccattgtatagcctgt

SEQ ID NO: 14848 - RNA, 20 nt, synthetic construct
  source 1..20: mol_type = other RNA
agcaagctagagggtgacag

SEQ ID NO: 14849 - RNA, 20 nt, synthetic construct
  source 1..20: mol_type = other RNA
tgggagcttagcaagctaga

SEQ ID NO: 14850 - RNA, 20 nt, synthetic construct
  source 1..20: mol_type = other RNA
ttgggagcttagcaagctag

SEQ ID NO: 14851 - RNA, 20 nt, synthetic construct
  source 1..20: mol_type = other RNA
acagcactagcacagtgcct

SEQ ID NO: 14852 - RNA, 20 nt, synthetic construct
  source 1..20: mol_type = other RNA
ggcactgtgctagtgctgtt

SEQ ID NO: 14853 - RNA, 20 nt, synthetic construct
  source 1..20: mol_type = other RNA
aggcactgtgctagtgctgt

SEQ ID NO: 14854 - RNA, 20 nt, synthetic construct
  source 1..20: mol_type = other RNA
agaggaaatcgcaggtacca

SEQ ID NO: 14855 - RNA, 20 nt, synthetic construct
  source 1..20: mol_type = other RNA
tgcgatttcctctacccaga

SEQ ID NO: 14856 - RNA, 20 nt, synthetic construct
  source 1..20: mol_type = other RNA
ttctgggtagaggaaatcgc

SEQ ID NO: 14857 - RNA, 20 nt, synthetic construct
  source 1..20: mol_type = other RNA
agaaggaaccttctgggtag

SEQ ID NO: 14858 - RNA, 20 nt, synthetic construct
  source 1..20: mol_type = other RNA
caaaaaagaaggaaccttct

SEQ ID NO: 14859 - RNA, 20 nt, synthetic construct
  source 1..20: mol_type = other RNA
acaaaaaagaaggaaccttc

SEQ ID NO: 14860 - RNA, 20 nt, synthetic construct
  source 1..20: mol_type = other RNA
tgtctcaaaaacaaaaaaga

SEQ ID NO: 14861 - RNA, 20 nt, synthetic construct
  source 1..20: mol_type = other RNA
cagtttcgctcttgttgccc

SEQ ID NO: 14862 - RNA, 20 nt, synthetic construct
  source 1..20: mol_type = other RNA
ttcgctcttgttgcccaggc

SEQ ID NO: 14863 - RNA, 20 nt, synthetic construct
  source 1..20: mol_type = other RNA
ttgcccaggctggagtgcaa

SEQ ID NO: 14864 - RNA, 20 nt, synthetic construct
  source 1..20: mol_type = other RNA
gcgccattgcactccagcct

SEQ ID NO: 14865 - RNA, 20 nt, synthetic construct
  source 1..20: mol_type = other RNA
cgcgccattgcactccagcc

SEQ ID NO: 14866 - RNA, 20 nt, synthetic construct
  source 1..20: mol_type = other RNA
ggagtgcaatggcgcgatct

SEQ ID NO: 14867 - RNA, 20 nt, synthetic construct
  source 1..20: mol_type = other RNA
aacgcaggaggtggagattg

SEQ ID NO: 14868 - RNA, 20 nt, synthetic construct
  source 1..20: mol_type = other RNA
aatcgcttgaacgcaggagg

SEQ ID NO: 14869 - RNA, 20 nt, synthetic construct
  source 1..20: mol_type = other RNA
gagaatcgcttgaacgcagg

SEQ ID NO: 14870 - RNA, 20 nt, synthetic construct
  source 1..20: mol_type = other RNA
caggagaatcgcttgaacgc

SEQ ID NO: 14871 - RNA, 20 nt, synthetic construct
  source 1..20: mol_type = other RNA
gcctcagcctcccaagtagc

SEQ ID NO: 14872 - RNA, 20 nt, synthetic construct
  source 1..20: mol_type = other RNA
cctcagcctcccaagtagct

SEQ ID NO: 14873 - RNA, 20 nt, synthetic construct
  source 1..20: mol_type = other RNA
gctacttgggaggctgaggc

SEQ ID NO: 14874 - RNA, 20 nt, synthetic construct
  source 1..20: mol_type = other RNA
cccagctacttgggaggctg

SEQ ID NO: 14875 - RNA, 20 nt, synthetic construct
  source 1..20: mol_type = other RNA
tcccaagtagctgggattac

SEQ ID NO: 14876 - RNA, 20 nt, synthetic construct
  source 1..20: mol_type = other RNA
tgtaatcccagctacttggg

SEQ ID NO: 14877 - RNA, 20 nt, synthetic construct
  source 1..20: mol_type = other RNA
gcctgtaatcccagctactt

SEQ ID NO: 14878 - RNA, 20 nt, synthetic construct
  source 1..20: mol_type = other RNA
tgcctgtaatcccagctact

SEQ ID NO: 14879 - RNA, 20 nt, synthetic construct
  source 1..20: mol_type = other RNA
acaaaattatctgggcatgg

SEQ ID NO: 14880 - RNA, 20 nt, synthetic construct
  source 1..20: mol_type = other RNA
aatacaaaattatctgggca

SEQ ID NO: 14881 - RNA, 20 nt, synthetic construct
  source 1..20: mol_type = other RNA
ctaaaaatacaaaattatct

SEQ ID NO: 14882 - RNA, 20 nt, synthetic construct
  source 1..20: mol_type = other RNA
actaaaaatacaaaattatc

SEQ ID NO: 14883 - RNA, 20 nt, synthetic construct
  source 1..20: mol_type = other RNA
tttgtatttttagtagagac

SEQ ID NO: 14884 - RNA, 20 nt, synthetic construct
  source 1..20: mol_type = other RNA
ttgtatttttagtagagaca

SEQ ID NO: 14885 - RNA, 20 nt, synthetic construct
  source 1..20: mol_type = other RNA
gagacagggcttcaccatgt

SEQ ID NO: 14886 - RNA, 20 nt, synthetic construct
  source 1..20: mol_type = other RNA
gcttcaccatgttggtcaga

SEQ ID NO: 14887 - RNA, 20 nt, synthetic construct
  source 1..20: mol_type = other RNA
tgagagccgtctgaccaaca

SEQ ID NO: 14888 - RNA, 20 nt, synthetic construct
  source 1..20: mol_type = other RNA
gtgcatcacttgaggtcaag

SEQ ID NO: 14889 - RNA, 20 nt, synthetic construct
  source 1..20: mol_type = other RNA
agaggtgggtgcatcacttg

SEQ ID NO: 14890 - RNA, 20 nt, synthetic construct
  source 1..20: mol_type = other RNA
acctctgcctcccaaagtgc

SEQ ID NO: 14891 - RNA, 20 nt, synthetic construct
  source 1..20: mol_type = other RNA
cctctgcctcccaaagtgct

SEQ ID NO: 14892 - RNA, 20 nt, synthetic construct
  source 1..20: mol_type = other RNA
gcactttgggaggcagaggt

SEQ ID NO: 14893 - RNA, 20 nt, synthetic construct
  source 1..20: mol_type = other RNA
agcactttgggaggcagagg

SEQ ID NO: 14894 - RNA, 20 nt, synthetic construct
  source 1..20: mol_type = other RNA
cccagcactttgggaggcag

SEQ ID NO: 14895 - RNA, 20 nt, synthetic construct
  source 1..20: mol_type = other RNA
tgtaatcccagcactttggg

SEQ ID NO: 14896 - RNA, 20 nt, synthetic construct
  source 1..20: mol_type = other RNA
gcttgtaatcccagcacttt

SEQ ID NO: 14897 - RNA, 20 nt, synthetic construct
  source 1..20: mol_type = other RNA
cgcttgtaatcccagcactt

SEQ ID NO: 14898 - RNA, 20 nt, synthetic construct
  source 1..20: mol_type = other RNA
caagcgtgagccaccgcgcc

SEQ ID NO: 14899 - RNA, 20 nt, synthetic construct
  source 1..20: mol_type = other RNA
caccgcgcctggcctccaga

SEQ ID NO: 14900 - RNA, 20 nt, synthetic construct
  source 1..20: mol_type = other RNA
cttctggaggccaggcgcgg

SEQ ID NO: 14901 - RNA, 20 nt, synthetic construct
  source 1..20: mol_type = other RNA
aaccttctggaggccaggcg

SEQ ID NO: 14902 - RNA, 20 nt, synthetic construct
  source 1..20: mol_type = other RNA
gaaggaaccttctggaggcc

SEQ ID NO: 14903 - RNA, 20 nt, synthetic construct
  source 1..20: mol_type = other RNA
ctccagaaggttccttctat

SEQ ID NO: 14904 - RNA, 20 nt, synthetic construct
  source 1..20: mol_type = other RNA
ctatagaaggaaccttctgg

SEQ ID NO: 14905 - RNA, 20 nt, synthetic construct
  source 1..20: mol_type = other RNA
agcctatagaaggaaccttc

SEQ ID NO: 14906 - RNA, 20 nt, synthetic construct
  source 1..20: mol_type = other RNA
cgctatgtgaagcctataga

SEQ ID NO: 14907 - RNA, 20 nt, synthetic construct
  source 1..20: mol_type = other RNA
gcgtgctccttcttgtcatt

SEQ ID NO: 14908 - RNA, 20 nt, synthetic construct
  source 1..20: mol_type = other RNA
ctgagatccaaatgacaaga

SEQ ID NO: 14909 - RNA, 20 nt, synthetic construct
  source 1..20: mol_type = other RNA
acctgctcagtaaagccttc

SEQ ID NO: 14910 - RNA, 20 nt, synthetic construct
  source 1..20: mol_type = other RNA
tccagaaggctttactgagc

SEQ ID NO: 14911 - RNA, 20 nt, synthetic construct
  source 1..20: mol_type = other RNA
attaagaaggacgctccaga

SEQ ID NO: 14912 - RNA, 20 nt, synthetic construct
  source 1..20: mol_type = other RNA
taggagactggggattaaga

SEQ ID NO: 14913 - RNA, 20 nt, synthetic construct
  source 1..20: mol_type = other RNA
tgaaacaggataggagactg

SEQ ID NO: 14914 - RNA, 20 nt, synthetic construct
  source 1..20: mol_type = other RNA
gtgaaacaggataggagact

SEQ ID NO: 14915 - RNA, 20 nt, synthetic construct
  source 1..20: mol_type = other RNA
agtgaaacaggataggagac

SEQ ID NO: 14916 - RNA, 20 nt, synthetic construct
  source 1..20: mol_type = other RNA
atcctgtttcacttcccgca

SEQ ID NO: 14917 - RNA, 20 nt, synthetic construct
  source 1..20: mol_type = other RNA
tgcgggaagtgaaacaggat

SEQ ID NO: 14918 - RNA, 20 nt, synthetic construct
  source 1..20: mol_type = other RNA
tgccatgcgggaagtgaaac

SEQ ID NO: 14919 - RNA, 20 nt, synthetic construct
  source 1..20: mol_type = other RNA
tagagtcacatgtgccatgc

SEQ ID NO: 14920 - RNA, 20 nt, synthetic construct
  source 1..20: mol_type = other RNA
ttagagtcacatgtgccatg

SEQ ID NO: 14921 - RNA, 20 nt, synthetic construct
  source 1..20: mol_type = other RNA
ttattttttataagtgtctg

SEQ ID NO: 14922 - RNA, 20 nt, synthetic construct
  source 1..20: mol_type = other RNA
tgtggaagtctgcattctag

SEQ ID NO: 14923 - RNA, 20 nt, synthetic construct
  source 1..20: mol_type = other RNA
atgcagacttccacagagca

SEQ ID NO: 14924 - RNA, 20 nt, synthetic construct
  source 1..20: mol_type = other RNA
aaggtaggggccttgctctg

SEQ ID NO: 14925 - RNA, 20 nt, synthetic construct
  source 1..20: mol_type = other RNA
gtgatcattgagaaaggtag

SEQ ID NO: 14926 - RNA, 20 nt, synthetic construct
  source 1..20: mol_type = other RNA
agtgatcattgagaaaggta

SEQ ID NO: 14927 - RNA, 20 nt, synthetic construct
  source 1..20: mol_type = other RNA
cagtgatcattgagaaaggt

SEQ ID NO: 14928 - RNA, 20 nt, synthetic construct
  source 1..20: mol_type = other RNA
gatacagtgatcattgagaa

SEQ ID NO: 14929 - RNA, 20 nt, synthetic construct
  source 1..20: mol_type = other RNA
taacaggtgttgtagacgct

SEQ ID NO: 14930 - RNA, 20 nt, synthetic construct
  source 1..20: mol_type = other RNA
gtctacaacacctgttacac

SEQ ID NO: 14931 - RNA, 20 nt, synthetic construct
  source 1..20: mol_type = other RNA
ttgatgacaacctgtgtaac

SEQ ID NO: 14932 - RNA, 20 nt, synthetic construct
  source 1..20: mol_type = other RNA
ttgtcatcaatgcacatgta

SEQ ID NO: 14933 - RNA, 20 nt, synthetic construct
  source 1..20: mol_type = other RNA
gaaaaaaagatcgaaagaga

SEQ ID NO: 14934 - RNA, 20 nt, synthetic construct
  source 1..20: mol_type = other RNA
aaaaaaagatcgaaagagat

SEQ ID NO: 14935 - RNA, 20 nt, synthetic construct
  source 1..20: mol_type = other RNA
aaagatcgaaagagatggga

SEQ ID NO: 14936 - RNA, 20 nt, synthetic construct
  source 1..20: mol_type = other RNA
caaaaaacacaagaaactcc

SEQ ID NO: 14937 - RNA, 20 nt, synthetic construct
  source 1..20: mol_type = other RNA
cggaaataattcaaattgcc

SEQ ID NO: 14938 - RNA, 20 nt, synthetic construct
  source 1..20: mol_type = other RNA
cggaaactgaggtgcaggag

SEQ ID NO: 14939 - RNA, 20 nt, synthetic construct
  source 1..20: mol_type = other RNA
agaggcggaaactgaggtgc

SEQ ID NO: 14940 - RNA, 20 nt, synthetic construct
  source 1..20: mol_type = other RNA
cagtttccgcctctgtaaaa

SEQ ID NO: 14941 - RNA, 20 nt, synthetic construct
  source 1..20: mol_type = other RNA
agtttccgcctctgtaaaat

SEQ ID NO: 14942 - RNA, 20 nt, synthetic construct
  source 1..20: mol_type = other RNA
ttttacagaggcggaaactg

SEQ ID NO: 14943 - RNA, 20 nt, synthetic construct
  source 1..20: mol_type = other RNA
gcgagcccattttacagagg

SEQ ID NO: 14944 - RNA, 20 nt, synthetic construct
  source 1..20: mol_type = other RNA
agcgcgagcccattttacag

SEQ ID NO: 14945 - RNA, 20 nt, synthetic construct
  source 1..20: mol_type = other RNA
gggcgggcggaggagggtta

SEQ ID NO: 14946 - RNA, 20 nt, synthetic construct
  source 1..20: mol_type = other RNA
cagagtgggcgggcggagga

SEQ ID NO: 14947 - RNA, 20 nt, synthetic construct
  source 1..20: mol_type = other RNA
tcagagtgggcgggcggagg

SEQ ID NO: 14948 - RNA, 20 nt, synthetic construct
  source 1..20: mol_type = other RNA
gtgtcagagtgggcgggcgg

SEQ ID NO: 14949 - RNA, 20 nt, synthetic construct
  source 1..20: mol_type = other RNA
cccgcccactctgacaccac

SEQ ID NO: 14950 - RNA, 20 nt, synthetic construct
  source 1..20: mol_type = other RNA
gtggtgtcagagtgggcggg

SEQ ID NO: 14951 - RNA, 20 nt, synthetic construct
  source 1..20: mol_type = other RNA
ccactctgacaccaccggaa

SEQ ID NO: 14952 - RNA, 20 nt, synthetic construct
  source 1..20: mol_type = other RNA
tccggtggtgtcagagtggg

SEQ ID NO: 14953 - RNA, 20 nt, synthetic construct
  source 1..20: mol_type = other RNA
ctttccggtggtgtcagagt

SEQ ID NO: 14954 - RNA, 20 nt, synthetic construct
  source 1..20: mol_type = other RNA
cctttccggtggtgtcagag

SEQ ID NO: 14955 - RNA, 20 nt, synthetic construct
  source 1..20: mol_type = other RNA
accaccggaaaggattcatt

SEQ ID NO: 14956 - RNA, 20 nt, synthetic construct
  source 1..20: mol_type = other RNA
ccaccggaaaggattcattc

SEQ ID NO: 14957 - RNA, 20 nt, synthetic construct
  source 1..20: mol_type = other RNA
cccgaatgaatcctttccgg

SEQ ID NO: 14958 - RNA, 20 nt, synthetic construct
  source 1..20: mol_type = other RNA
gttcccgaatgaatcctttc

SEQ ID NO: 14959 - RNA, 20 nt, synthetic construct
  source 1..20: mol_type = other RNA
gattcattcgggaacattcg

SEQ ID NO: 14960 - RNA, 20 nt, synthetic construct
  source 1..20: mol_type = other RNA
attcattcgggaacattcgt

SEQ ID NO: 14961 - RNA, 20 nt, synthetic construct
  source 1..20: mol_type = other RNA
ttcattcgggaacattcgtg

SEQ ID NO: 14962 - RNA, 20 nt, synthetic construct
  source 1..20: mol_type = other RNA
attcgggaacattcgtgggg

SEQ ID NO: 14963 - RNA, 20 nt, synthetic construct
  source 1..20: mol_type = other RNA
gaacattcgtggggcggaga

SEQ ID NO: 14964 - RNA, 20 nt, synthetic construct
  source 1..20: mol_type = other RNA
aacattcgtggggcggagac

SEQ ID NO: 14965 - RNA, 20 nt, synthetic construct
  source 1..20: mol_type = other RNA
tcgtggggcggagacgggac

SEQ ID NO: 14966 - RNA, 20 nt, synthetic construct
  source 1..20: mol_type = other RNA
cgtggggcggagacgggaca

SEQ ID NO: 14967 - RNA, 20 nt, synthetic construct
  source 1..20: mol_type = other RNA
gtggggcggagacgggacag

SEQ ID NO: 14968 - RNA, 20 nt, synthetic construct
  source 1..20: mol_type = other RNA
tggggcggagacgggacagg

SEQ ID NO: 14969 - RNA, 20 nt, synthetic construct
  source 1..20: mol_type = other RNA
ggagacgggacagggggcct

SEQ ID NO: 14970 - RNA, 20 nt, synthetic construct
  source 1..20: mol_type = other RNA
ggacgtgacgctacaggccg

SEQ ID NO: 14971 - RNA, 20 nt, synthetic construct
  source 1..20: mol_type = other RNA
cctgtagcgtcacgtccgcc

SEQ ID NO: 14972 - RNA, 20 nt, synthetic construct
  source 1..20: mol_type = other RNA
ctgtagcgtcacgtccgcca

SEQ ID NO: 14973 - RNA, 20 nt, synthetic construct
  source 1..20: mol_type = other RNA
cctggcggacgtgacgctac

SEQ ID NO: 14974 - RNA, 20 nt, synthetic construct
  source 1..20: mol_type = other RNA
acgtccgccagggttacctg

SEQ ID NO: 14975 - RNA, 20 nt, synthetic construct
  source 1..20: mol_type = other RNA
cgtccgccagggttacctgt

SEQ ID NO: 14976 - RNA, 20 nt, synthetic construct
  source 1..20: mol_type = other RNA
gtccgccagggttacctgtg

SEQ ID NO: 14977 - RNA, 20 nt, synthetic construct
  source 1..20: mol_type = other RNA
gccagggttacctgtggggc

SEQ ID NO: 14978 - RNA, 20 nt, synthetic construct
  source 1..20: mol_type = other RNA
ccagggttacctgtggggct

SEQ ID NO: 14979 - RNA, 20 nt, synthetic construct
  source 1..20: mol_type = other RNA
agccccacaggtaaccctgg

SEQ ID NO: 14980 - RNA, 20 nt, synthetic construct
  source 1..20: mol_type = other RNA
cccagccccacaggtaaccc

SEQ ID NO: 14981 - RNA, 20 nt, synthetic construct
  source 1..20: mol_type = other RNA
cggttcgctcccagccccac

SEQ ID NO: 14982 - RNA, 20 nt, synthetic construct
  source 1..20: mol_type = other RNA
ccgcactcgcaccgcaaccc

SEQ ID NO: 14983 - RNA, 20 nt, synthetic construct
  source 1..20: mol_type = other RNA
ccggggttgcggtgcgagtg

SEQ ID NO: 14984 - RNA, 20 nt, synthetic construct
  source 1..20: mol_type = other RNA
caaccccggcatcagtgccc

SEQ ID NO: 14985 - RNA, 20 nt, synthetic construct
  source 1..20: mol_type = other RNA
gggcactgatgccggggttg

SEQ ID NO: 14986 - RNA, 20 nt, synthetic construct
  source 1..20: mol_type = other RNA
cccggcatcagtgcccaggt

SEQ ID NO: 14987 - RNA, 20 nt, synthetic construct
  source 1..20: mol_type = other RNA
caacctgggcactgatgccg

SEQ ID NO: 14988 - RNA, 20 nt, synthetic construct
  source 1..20: mol_type = other RNA
ccaacctgggcactgatgcc

SEQ ID NO: 14989 - RNA, 20 nt, synthetic construct
  source 1..20: mol_type = other RNA
gccaacctgggcactgatgc

SEQ ID NO: 14990 - RNA, 20 nt, synthetic construct
  source 1..20: mol_type = other RNA
ggacggcgcgaggccaacct

SEQ ID NO: 14991 - RNA, 20 nt, synthetic construct
  source 1..20: mol_type = other RNA
aggacggcgcgaggccaacc

SEQ ID NO: 14992 - RNA, 20 nt, synthetic construct
  source 1..20: mol_type = other RNA
tggcctcgcgccgtcctacg

SEQ ID NO: 14993 - RNA, 20 nt, synthetic construct
  source 1..20: mol_type = other RNA
cctcgcgccgtcctacgggg

SEQ ID NO: 14994 - RNA, 20 nt, synthetic construct
  source 1..20: mol_type = other RNA
ccgccccgtaggacggcgcg

SEQ ID NO: 14995 - RNA, 20 nt, synthetic construct
  source 1..20: mol_type = other RNA
ccgtcctacggggcggccag

SEQ ID NO: 14996 - RNA, 20 nt, synthetic construct
  source 1..20: mol_type = other RNA
cctctggccgccccgtagga

SEQ ID NO: 14997 - RNA, 20 nt, synthetic construct
  source 1..20: mol_type = other RNA
gcggcctctggccgccccgt

SEQ ID NO: 14998 - RNA, 20 nt, synthetic construct
  source 1..20: mol_type = other RNA
gggcggccagaggccgccga

SEQ ID NO: 14999 - RNA, 20 nt, synthetic construct
  source 1..20: mol_type = other RNA
gagaggccttcggcggcctc

SEQ ID NO: 15000 - RNA, 20 nt, synthetic construct
  source 1..20: mol_type = other RNA
gcagcgcgagaggccttcgg

SEQ ID NO: 15001 - RNA, 20 nt, synthetic construct
  source 1..20: mol_type = other RNA
gctgcagcgcgagaggcctt

SEQ ID NO: 15002 - RNA, 20 nt, synthetic construct
  source 1..20: mol_type = other RNA
ggagactgctgcagcgcgag

SEQ ID NO: 15003 - RNA, 20 nt, synthetic construct
  source 1..20: mol_type = other RNA
tcctcaggagcgccgccatg

SEQ ID NO: 15004 - RNA, 20 nt, synthetic construct
  source 1..20: mol_type = other RNA
cctcaggagcgccgccatgt

SEQ ID NO: 15005 - RNA, 20 nt, synthetic construct
  source 1..20: mol_type = other RNA
aggagcgccgccatgtggga

SEQ ID NO: 15006 - RNA, 20 nt, synthetic construct
  source 1..20: mol_type = other RNA
cccacatggcggcgctcctg

SEQ ID NO: 15007 - RNA, 20 nt, synthetic construct
  source 1..20: mol_type = other RNA
tgctattccatcccacatgg

SEQ ID NO: 15008 - RNA, 20 nt, synthetic construct
  source 1..20: mol_type = other RNA
gtgggatggaatagcacacg

SEQ ID NO: 15009 - RNA, 20 nt, synthetic construct
  source 1..20: mol_type = other RNA
gtgtgctattccatcccaca

SEQ ID NO: 15010 - RNA, 20 nt, synthetic construct
  source 1..20: mol_type = other RNA
gcttctccctgcgtcacttc

SEQ ID NO: 15011 - RNA, 20 nt, synthetic construct
  source 1..20: mol_type = other RNA
cttctccctgcgtcacttcc

SEQ ID NO: 15012 - RNA, 20 nt, synthetic construct
  source 1..20: mol_type = other RNA
ttctccctgcgtcacttccg

SEQ ID NO: 15013 - RNA, 20 nt, synthetic construct
  source 1..20: mol_type = other RNA
cagtccccggaagtgacgca

SEQ ID NO: 15014 - RNA, 20 nt, synthetic construct
  source 1..20: mol_type = other RNA
gcagtccccggaagtgacgc

SEQ ID NO: 15015 - RNA, 20 nt, synthetic construct
  source 1..20: mol_type = other RNA
ggggactgcttccagccaat

SEQ ID NO: 15016 - RNA, 20 nt, synthetic construct
  source 1..20: mol_type = other RNA
gattggctggaagcagtccc

SEQ ID NO: 15017 - RNA, 20 nt, synthetic construct
  source 1..20: mol_type = other RNA
tgtggcggaggccgattggc

SEQ ID NO: 15018 - RNA, 20 nt, synthetic construct
  source 1..20: mol_type = other RNA
tggctgtggcggaggccgat

SEQ ID NO: 15019 - RNA, 20 nt, synthetic construct
  source 1..20: mol_type = other RNA
ggctgcgctggctgtggcgg

SEQ ID NO: 15020 - RNA, 20 nt, synthetic construct
  source 1..20: mol_type = other RNA
caaggctgcgctggctgtgg

SEQ ID NO: 15021 - RNA, 20 nt, synthetic construct
  source 1..20: mol_type = other RNA
gggcaaggctgcgctggctg

SEQ ID NO: 15022 - RNA, 20 nt, synthetic construct
  source 1..20: mol_type = other RNA
tttaaggggcaaggctgcgc

SEQ ID NO: 15023 - RNA, 20 nt, synthetic construct
  source 1..20: mol_type = other RNA
gccttgccccttaaagtcac

SEQ ID NO: 15024 - RNA, 20 nt, synthetic construct
  source 1..20: mol_type = other RNA
gcctgtgactttaaggggca

SEQ ID NO: 15025 - RNA, 20 nt, synthetic construct
  source 1..20: mol_type = other RNA
agggggcctgtgactttaag

SEQ ID NO: 15026 - RNA, 20 nt, synthetic construct
  source 1..20: mol_type = other RNA
tagggggcctgtgactttaa

SEQ ID NO: 15027 - RNA, 20 nt, synthetic construct
  source 1..20: mol_type = other RNA
ctagggggcctgtgacttta

SEQ ID NO: 15028 - RNA, 20 nt, synthetic construct
  source 1..20: mol_type = other RNA
gcgtgggatttcgcgctagg

SEQ ID NO: 15029 - RNA, 20 nt, synthetic construct
  source 1..20: mol_type = other RNA
ggcgtgggatttcgcgctag

SEQ ID NO: 15030 - RNA, 20 nt, synthetic construct
  source 1..20: mol_type = other RNA
gggcgtgggatttcgcgcta

SEQ ID NO: 15031 - RNA, 20 nt, synthetic construct
  source 1..20: mol_type = other RNA
ggggcgtgggatttcgcgct

SEQ ID NO: 15032 - RNA, 20 nt, synthetic construct
  source 1..20: mol_type = other RNA
aaatcccacgcccccctgga

SEQ ID NO: 15033 - RNA, 20 nt, synthetic construct
  source 1..20: mol_type = other RNA
cacgcccccctggacggctg

SEQ ID NO: 15034 - RNA, 20 nt, synthetic construct
  source 1..20: mol_type = other RNA
gcagccgtccaggggggcgt

SEQ ID NO: 15035 - RNA, 20 nt, synthetic construct
  source 1..20: mol_type = other RNA
cgcagccgtccaggggggcg

SEQ ID NO: 15036 - RNA, 20 nt, synthetic construct
  source 1..20: mol_type = other RNA
gcggccgcagccgtccaggg

SEQ ID NO: 15037 - RNA, 20 nt, synthetic construct
  source 1..20: mol_type = other RNA
tgcggccgcagccgtccagg

SEQ ID NO: 15038 - RNA, 20 nt, synthetic construct
  source 1..20: mol_type = other RNA
gtgcggccgcagccgtccag

SEQ ID NO: 15039 - RNA, 20 nt, synthetic construct
  source 1..20: mol_type = other RNA
agtgcggccgcagccgtcca

SEQ ID NO: 15040 - RNA, 20 nt, synthetic construct
  source 1..20: mol_type = other RNA
gagtgcggccgcagccgtcc

SEQ ID NO: 15041 - RNA, 20 nt, synthetic construct
  source 1..20: mol_type = other RNA
ctgcggccgcactcgccacc

SEQ ID NO: 15042 - RNA, 20 nt, synthetic construct
  source 1..20: mol_type = other RNA
tgcggccgcactcgccacca

SEQ ID NO: 15043 - RNA, 20 nt, synthetic construct
  source 1..20: mol_type = other RNA
gcggccgcactcgccaccag

SEQ ID NO: 15044 - RNA, 20 nt, synthetic construct
  source 1..20: mol_type = other RNA
cggccgcactcgccaccagg

SEQ ID NO: 15045 - RNA, 20 nt, synthetic construct
  source 1..20: mol_type = other RNA
cactcgccaccagggggcag

SEQ ID NO: 15046 - RNA, 20 nt, synthetic construct
  source 1..20: mol_type = other RNA
ctgccccctggtggcgagtg

SEQ ID NO: 15047 - RNA, 20 nt, synthetic construct
  source 1..20: mol_type = other RNA
agggggcagaggccagagaa

SEQ ID NO: 15048 - RNA, 20 nt, synthetic construct
  source 1..20: mol_type = other RNA
gggggcagaggccagagaaa

SEQ ID NO: 15049 - RNA, 20 nt, synthetic construct
  source 1..20: mol_type = other RNA
tttctctggcctctgccccc

SEQ ID NO: 15050 - RNA, 20 nt, synthetic construct
  source 1..20: mol_type = other RNA
ccagagaaagggctatttcc

SEQ ID NO: 15051 - RNA, 20 nt, synthetic construct
  source 1..20: mol_type = other RNA
ccgggaaatagccctttctc

SEQ ID NO: 15052 - RNA, 20 nt, synthetic construct
  source 1..20: mol_type = other RNA
cggacccgcccccttcagct

SEQ ID NO: 15053 - RNA, 20 nt, synthetic construct
  source 1..20: mol_type = other RNA
ggacccgcccccttcagctt

SEQ ID NO: 15054 - RNA, 20 nt, synthetic construct
  source 1..20: mol_type = other RNA
aagctgaagggggcgggtcc

SEQ ID NO: 15055 - RNA, 20 nt, synthetic construct
  source 1..20: mol_type = other RNA
caagctgaagggggcgggtc

SEQ ID NO: 15056 - RNA, 20 nt, synthetic construct
  source 1..20: mol_type = other RNA
tttcccaagctgaagggggc

SEQ ID NO: 15057 - RNA, 20 nt, synthetic construct
  source 1..20: mol_type = other RNA
ctttcccaagctgaaggggg

SEQ ID NO: 15058 - RNA, 20 nt, synthetic construct
  source 1..20: mol_type = other RNA
tcgctttcccaagctgaagg

SEQ ID NO: 15059 - RNA, 20 nt, synthetic construct
  source 1..20: mol_type = other RNA
ttcgctttcccaagctgaag

SEQ ID NO: 15060 - RNA, 20 nt, synthetic construct
  source 1..20: mol_type = other RNA
tttcgctttcccaagctgaa

SEQ ID NO: 15061 - RNA, 20 nt, synthetic construct
  source 1..20: mol_type = other RNA
agcttgggaaagcgaaagcg

SEQ ID NO: 15062 - RNA, 20 nt, synthetic construct
  source 1..20: mol_type = other RNA
tgggaaagcgaaagcgtggc

SEQ ID NO: 15063 - RNA, 20 nt, synthetic construct
  source 1..20: mol_type = other RNA
gggaaagcgaaagcgtggca

SEQ ID NO: 15064 - RNA, 20 nt, synthetic construct
  source 1..20: mol_type = other RNA
ggaaagcgaaagcgtggcag

SEQ ID NO: 15065 - RNA, 20 nt, synthetic construct
  source 1..20: mol_type = other RNA
agcgaaagcgtggcaggggc

SEQ ID NO: 15066 - RNA, 20 nt, synthetic construct
  source 1..20: mol_type = other RNA
agcgtggcaggggccggacc

SEQ ID NO: 15067 - RNA, 20 nt, synthetic construct
  source 1..20: mol_type = other RNA
gcgtggcaggggccggacct

SEQ ID NO: 15068 - RNA, 20 nt, synthetic construct
  source 1..20: mol_type = other RNA
gcaggggccggacctgggag

SEQ ID NO: 15069 - RNA, 20 nt, synthetic construct
  source 1..20: mol_type = other RNA
ggggccggacctgggagcgg

SEQ ID NO: 15070 - RNA, 20 nt, synthetic construct
  source 1..20: mol_type = other RNA
gccggacctgggagcggagg

SEQ ID NO: 15071 - RNA, 20 nt, synthetic construct
  source 1..20: mol_type = other RNA
ggacctgggagcggaggagg

SEQ ID NO: 15072 - RNA, 20 nt, synthetic construct
  source 1..20: mol_type = other RNA
gacctgggagcggaggaggc

SEQ ID NO: 15073 - RNA, 20 nt, synthetic construct
  source 1..20: mol_type = other RNA
gcctcctccgctcccaggtc

SEQ ID NO: 15074 - RNA, 20 nt, synthetic construct
  source 1..20: mol_type = other RNA
gacccgcctcctccgctccc

SEQ ID NO: 15075 - RNA, 20 nt, synthetic construct
  source 1..20: mol_type = other RNA
tagaaacctccacctgtttc

SEQ ID NO: 15076 - RNA, 20 nt, synthetic construct
  source 1..20: mol_type = other RNA
gaaacaggtggaggtttcta

SEQ ID NO: 15077 - RNA, 20 nt, synthetic construct
  source 1..20: mol_type = other RNA
aacctccacctgtttccggc

SEQ ID NO: 15078 - RNA, 20 nt, synthetic construct
  source 1..20: mol_type = other RNA
acctccacctgtttccggcc

SEQ ID NO: 15079 - RNA, 20 nt, synthetic construct
  source 1..20: mol_type = other RNA
gcccggccggaaacaggtgg

SEQ ID NO: 15080 - RNA, 20 nt, synthetic construct
  source 1..20: mol_type = other RNA
acagcccggccggaaacagg

SEQ ID NO: 15081 - RNA, 20 nt, synthetic construct
  source 1..20: mol_type = other RNA
ctcacagcccggccggaaac

SEQ ID NO: 15082 - RNA, 20 nt, synthetic construct
  source 1..20: mol_type = other RNA
cggccgggctgtgagagatt

SEQ ID NO: 15083 - RNA, 20 nt, synthetic construct
  source 1..20: mol_type = other RNA
ggccgggctgtgagagatta

SEQ ID NO: 15084 - RNA, 20 nt, synthetic construct
  source 1..20: mol_type = other RNA
gccgggctgtgagagattag

SEQ ID NO: 15085 - RNA, 20 nt, synthetic construct
  source 1..20: mol_type = other RNA
ctaatctctcacagcccggc

SEQ ID NO: 15086 - RNA, 20 nt, synthetic construct
  source 1..20: mol_type = other RNA
gcccctaatctctcacagcc

SEQ ID NO: 15087 - RNA, 20 nt, synthetic construct
  source 1..20: mol_type = other RNA
tgagagattaggggctgctg

SEQ ID NO: 15088 - RNA, 20 nt, synthetic construct
  source 1..20: mol_type = other RNA
gagagattaggggctgctgc

SEQ ID NO: 15089 - RNA, 20 nt, synthetic construct
  source 1..20: mol_type = other RNA
agagattaggggctgctgcg

SEQ ID NO: 15090 - RNA, 20 nt, synthetic construct
  source 1..20: mol_type = other RNA
gagattaggggctgctgcgg

SEQ ID NO: 15091 - RNA, 20 nt, synthetic construct
  source 1..20: mol_type = other RNA
agaggcgagctggctgagat

SEQ ID NO: 15092 - RNA, 20 nt, synthetic construct
  source 1..20: mol_type = other RNA
gccagctcgcctcttcccag

SEQ ID NO: 15093 - RNA, 20 nt, synthetic construct
  source 1..20: mol_type = other RNA
gccgctgggaagaggcgagc

SEQ ID NO: 15094 - RNA, 20 nt, synthetic construct
  source 1..20: mol_type = other RNA
cctcttcccagcggcctctg

SEQ ID NO: 15095 - RNA, 20 nt, synthetic construct
  source 1..20: mol_type = other RNA
ctcttcccagcggcctctgc

SEQ ID NO: 15096 - RNA, 20 nt, synthetic construct
  source 1..20: mol_type = other RNA
ccgcagaggccgctgggaag

SEQ ID NO: 15097 - RNA, 20 nt, synthetic construct
  source 1..20: mol_type = other RNA
cccagcggcctctgcgggag

SEQ ID NO: 15098 - RNA, 20 nt, synthetic construct
  source 1..20: mol_type = other RNA
agcggcctctgcgggagcgg

SEQ ID NO: 15099 - RNA, 20 nt, synthetic construct
  source 1..20: mol_type = other RNA
gcggcctctgcgggagcggt

SEQ ID NO: 15100 - RNA, 20 nt, synthetic construct
  source 1..20: mol_type = other RNA
ccgctcccgcagaggccgct

SEQ ID NO: 15101 - RNA, 20 nt, synthetic construct
  source 1..20: mol_type = other RNA
accgctcccgcagaggccgc

SEQ ID NO: 15102 - RNA, 20 nt, synthetic construct
  source 1..20: mol_type = other RNA
aacacccaccgctcccgcag

SEQ ID NO: 15103 - RNA, 20 nt, synthetic construct
  source 1..20: mol_type = other RNA
ggtgttgtacacaatcatca

SEQ ID NO: 15104 - RNA, 20 nt, synthetic construct
  source 1..20: mol_type = other RNA
gttgtacacaatcatcatgg

SEQ ID NO: 15105 - RNA, 20 nt, synthetic construct
  source 1..20: mol_type = other RNA
gtacacaatcatcatggcgg

SEQ ID NO: 15106 - RNA, 20 nt, synthetic construct
  source 1..20: mol_type = other RNA
acaatcatcatggcggcggc

SEQ ID NO: 15107 - RNA, 20 nt, synthetic construct
  source 1..20: mol_type = other RNA
caatcatcatggcggcggcc

SEQ ID NO: 15108 - RNA, 20 nt, synthetic construct
  source 1..20: mol_type = other RNA
aatcatcatggcggcggccg

SEQ ID NO: 15109 - RNA, 20 nt, synthetic construct
  source 1..20: mol_type = other RNA
catggcggcggccggggccc

SEQ ID NO: 15110 - RNA, 20 nt, synthetic construct
  source 1..20: mol_type = other RNA
gcggcggccggggccccgga

SEQ ID NO: 15111 - RNA, 20 nt, synthetic construct
  source 1..20: mol_type = other RNA
ggggccccggatggtgagtg

SEQ ID NO: 15112 - RNA, 20 nt, synthetic construct
  source 1..20: mol_type = other RNA
gccccggatggtgagtgcgg

SEQ ID NO: 15113 - RNA, 20 nt, synthetic construct
  source 1..20: mol_type = other RNA
ccccggatggtgagtgcggc

SEQ ID NO: 15114 - RNA, 20 nt, synthetic construct
  source 1..20: mol_type = other RNA
cccggatggtgagtgcggcg

SEQ ID NO: 15115 - RNA, 20 nt, synthetic construct
  source 1..20: mol_type = other RNA
ccggatggtgagtgcggcgg

SEQ ID NO: 15116 - RNA, 20 nt, synthetic construct
  source 1..20: mol_type = other RNA
gatggtgagtgcggcggggg

SEQ ID NO: 15117 - RNA, 20 nt, synthetic construct
  source 1..20: mol_type = other RNA
ccccgccgcactcaccatcc

SEQ ID NO: 15118 - RNA, 20 nt, synthetic construct
  source 1..20: mol_type = other RNA
cccccgccgcactcaccatc

SEQ ID NO: 15119 - RNA, 20 nt, synthetic construct
  source 1..20: mol_type = other RNA
ggtgagtgcggcgggggtgg

SEQ ID NO: 15120 - RNA, 20 nt, synthetic construct
  source 1..20: mol_type = other RNA
gtgagtgcggcgggggtggc

SEQ ID NO: 15121 - RNA, 20 nt, synthetic construct
  source 1..20: mol_type = other RNA
gcggcgggggtggcgggcgc

SEQ ID NO: 15122 - RNA, 20 nt, synthetic construct
  source 1..20: mol_type = other RNA
cggcgggggtggcgggcgcc

SEQ ID NO: 15123 - RNA, 20 nt, synthetic construct
  source 1..20: mol_type = other RNA
gggggtggcgggcgccgggc

SEQ ID NO: 15124 - RNA, 20 nt, synthetic construct
  source 1..20: mol_type = other RNA
ggggtggcgggcgccgggcc

SEQ ID NO: 15125 - RNA, 20 nt, synthetic construct
  source 1..20: mol_type = other RNA
gggtggcgggcgccgggccg

SEQ ID NO: 15126 - RNA, 20 nt, synthetic construct
  source 1..20: mol_type = other RNA
cgggcgccgggccggggctg

SEQ ID NO: 15127 - RNA, 20 nt, synthetic construct
  source 1..20: mol_type = other RNA
ccgggccggggctgaggttg

SEQ ID NO: 15128 - RNA, 20 nt, synthetic construct
  source 1..20: mol_type = other RNA
ccgcaacctcagccccggcc

SEQ ID NO: 15129 - RNA, 20 nt, synthetic construct
  source 1..20: mol_type = other RNA
agcgaccgcaacctcagccc

SEQ ID NO: 15130 - RNA, 20 nt, synthetic construct
  source 1..20: mol_type = other RNA
tgaggttgcggtcgctcctc

SEQ ID NO: 15131 - RNA, 20 nt, synthetic construct
  source 1..20: mol_type = other RNA
gaggttgcggtcgctcctct

SEQ ID NO: 15132 - RNA, 20 nt, synthetic construct
  source 1..20: mol_type = other RNA
aggttgcggtcgctcctctg

SEQ ID NO: 15133 - RNA, 20 nt, synthetic construct
  source 1..20: mol_type = other RNA
ggttgcggtcgctcctctgg

SEQ ID NO: 15134 - RNA, 20 nt, synthetic construct
  source 1..20: mol_type = other RNA
ggtcgctcctctgggggatg

SEQ ID NO: 15135 - RNA, 20 nt, synthetic construct
  source 1..20: mol_type = other RNA
ctcctctgggggatgcggcc

SEQ ID NO: 15136 - RNA, 20 nt, synthetic construct
  source 1..20: mol_type = other RNA
ctgggggatgcggcccggcc

SEQ ID NO: 15137 - RNA, 20 nt, synthetic construct
  source 1..20: mol_type = other RNA
tgggggatgcggcccggccc

SEQ ID NO: 15138 - RNA, 20 nt, synthetic construct
  source 1..20: mol_type = other RNA
ggccgggccgcatcccccag

SEQ ID NO: 15139 - RNA, 20 nt, synthetic construct
  source 1..20: mol_type = other RNA
gggatgcggcccggcccggg

SEQ ID NO: 15140 - RNA, 20 nt, synthetic construct
  source 1..20: mol_type = other RNA
ggatgcggcccggcccggga

SEQ ID NO: 15141 - RNA, 20 nt, synthetic construct
  source 1..20: mol_type = other RNA
cggcccgggagggagaaccg

SEQ ID NO: 15142 - RNA, 20 nt, synthetic construct
  source 1..20: mol_type = other RNA
gcggttctccctcccgggcc

SEQ ID NO: 15143 - RNA, 20 nt, synthetic construct
  source 1..20: mol_type = other RNA
cgcggttctccctcccgggc

SEQ ID NO: 15144 - RNA, 20 nt, synthetic construct
  source 1..20: mol_type = other RNA
cgggagggagaaccgcggct

SEQ ID NO: 15145 - RNA, 20 nt, synthetic construct
  source 1..20: mol_type = other RNA
gggagggagaaccgcggctc

SEQ ID NO: 15146 - RNA, 20 nt, synthetic construct
  source 1..20: mol_type = other RNA
gagccgcggttctccctccc

SEQ ID NO: 15147 - RNA, 20 nt, synthetic construct
  source 1..20: mol_type = other RNA
cgagccgcggttctccctcc

SEQ ID NO: 15148 - RNA, 20 nt, synthetic construct
  source 1..20: mol_type = other RNA
ggagaaccgcggctcgggaa

SEQ ID NO: 15149 - RNA, 20 nt, synthetic construct
  source 1..20: mol_type = other RNA
gaaccgcggctcgggaacgg

SEQ ID NO: 15150 - RNA, 20 nt, synthetic construct
  source 1..20: mol_type = other RNA
gcggctcgggaacggaggtc

SEQ ID NO: 15151 - RNA, 20 nt, synthetic construct
  source 1..20: mol_type = other RNA
gctcgggaacggaggtccgg

SEQ ID NO: 15152 - RNA, 20 nt, synthetic construct
  source 1..20: mol_type = other RNA
aacggaggtccggcggcgcc

SEQ ID NO: 15153 - RNA, 20 nt, synthetic construct
  source 1..20: mol_type = other RNA
ggacgctgtccgggcgccgc

SEQ ID NO: 15154 - RNA, 20 nt, synthetic construct
  source 1..20: mol_type = other RNA
cttgggaacggacgctgtcc

SEQ ID NO: 15155 - RNA, 20 nt, synthetic construct
  source 1..20: mol_type = other RNA
gcttgggaacggacgctgtc

SEQ ID NO: 15156 - RNA, 20 nt, synthetic construct
  source 1..20: mol_type = other RNA
ccgttcccaagcccagcccg

SEQ ID NO: 15157 - RNA, 20 nt, synthetic construct
  source 1..20: mol_type = other RNA
ccgcgggctgggcttgggaa

SEQ ID NO: 15158 - RNA, 20 nt, synthetic construct
  source 1..20: mol_type = other RNA
gctcgccgcgggctgggctt

SEQ ID NO: 15159 - RNA, 20 nt, synthetic construct
  source 1..20: mol_type = other RNA
cgctcgccgcgggctgggct

SEQ ID NO: 15160 - RNA, 20 nt, synthetic construct
  source 1..20: mol_type = other RNA
gtgggcgctcgccgcgggct

SEQ ID NO: 15161 - RNA, 20 nt, synthetic construct
  source 1..20: mol_type = other RNA
ggtgggcgctcgccgcgggc

SEQ ID NO: 15162 - RNA, 20 nt, synthetic construct
  source 1..20: mol_type = other RNA
agggggtgggcgctcgccgc

SEQ ID NO: 15163 - RNA, 20 nt, synthetic construct
  source 1..20: mol_type = other RNA
tagggggtgggcgctcgccg

SEQ ID NO: 15164 - RNA, 20 nt, synthetic construct
  source 1..20: mol_type = other RNA
ccaccccctaacccccttgc

SEQ ID NO: 15165 - RNA, 20 nt, synthetic construct
  source 1..20: mol_type = other RNA
ctgcaagggggttagggggt

SEQ ID NO: 15166 - RNA, 20 nt, synthetic construct
  source 1..20: mol_type = other RNA
cctgcaagggggttaggggg

SEQ ID NO: 15167 - RNA, 20 nt, synthetic construct
  source 1..20: mol_type = other RNA
atgcctgcaagggggttagg

SEQ ID NO: 15168 - RNA, 20 nt, synthetic construct
  source 1..20: mol_type = other RNA
catgcctgcaagggggttag

SEQ ID NO: 15169 - RNA, 20 nt, synthetic construct
  source 1..20: mol_type = other RNA
ccatgcctgcaagggggtta

SEQ ID NO: 15170 - RNA, 20 nt, synthetic construct
  source 1..20: mol_type = other RNA
tccatgcctgcaagggggtt

SEQ ID NO: 15171 - RNA, 20 nt, synthetic construct
  source 1..20: mol_type = other RNA
cttgcaggcatggaggaacc

SEQ ID NO: 15172 - RNA, 20 nt, synthetic construct
  source 1..20: mol_type = other RNA
gttcctccatgcctgcaagg

SEQ ID NO: 15173 - RNA, 20 nt, synthetic construct
  source 1..20: mol_type = other RNA
ggttcctccatgcctgcaag

SEQ ID NO: 15174 - RNA, 20 nt, synthetic construct
  source 1..20: mol_type = other RNA
aggttcctccatgcctgcaa

SEQ ID NO: 15175 - RNA, 20 nt, synthetic construct
  source 1..20: mol_type = other RNA
caggttcctccatgcctgca

SEQ ID NO: 15176 - RNA, 20 nt, synthetic construct
  source 1..20: mol_type = other RNA
aggcatggaggaacctggca

SEQ ID NO: 15177 - RNA, 20 nt, synthetic construct
  source 1..20: mol_type = other RNA
ggaggaacctggcatggaca

SEQ ID NO: 15178 - RNA, 20 nt, synthetic construct
  source 1..20: mol_type = other RNA
ggaacctggcatggacacgg

SEQ ID NO: 15179 - RNA, 20 nt, synthetic construct
  source 1..20: mol_type = other RNA
tcggcctccgtgtccatgcc

SEQ ID NO: 15180 - RNA, 20 nt, synthetic construct
  source 1..20: mol_type = other RNA
ggacacggaggccgagactg

SEQ ID NO: 15181 - RNA, 20 nt, synthetic construct
  source 1..20: mol_type = other RNA
ggccgagactgtggctactg

SEQ ID NO: 15182 - RNA, 20 nt, synthetic construct
  source 1..20: mol_type = other RNA
agcctcagtagccacagtct

SEQ ID NO: 15183 - RNA, 20 nt, synthetic construct
  source 1..20: mol_type = other RNA
tggctactgaggctcccgcg

SEQ ID NO: 15184 - RNA, 20 nt, synthetic construct
  source 1..20: mol_type = other RNA
cgcgcggcccgtcaactgcc

SEQ ID NO: 15185 - RNA, 20 nt, synthetic construct
  source 1..20: mol_type = other RNA
gcggcccgtcaactgcctgg

SEQ ID NO: 15186 - RNA, 20 nt, synthetic construct
  source 1..20: mol_type = other RNA
caggcagttgacgggccgcg

SEQ ID NO: 15187 - RNA, 20 nt, synthetic construct
  source 1..20: mol_type = other RNA
tcagcctccaggcagttgac

SEQ ID NO: 15188 - RNA, 20 nt, synthetic construct
  source 1..20: mol_type = other RNA
ttcagcctccaggcagttga

SEQ ID NO: 15189 - RNA, 20 nt, synthetic construct
  source 1..20: mol_type = other RNA
ctgcctggaggctgaagccg

SEQ ID NO: 15190 - RNA, 20 nt, synthetic construct
  source 1..20: mol_type = other RNA
cctggaggctgaagccgcgg

SEQ ID NO: 15191 - RNA, 20 nt, synthetic construct
  source 1..20: mol_type = other RNA
ctggaggctgaagccgcggc

SEQ ID NO: 15192 - RNA, 20 nt, synthetic construct
  source 1..20: mol_type = other RNA
tggaggctgaagccgcggcg

SEQ ID NO: 15193 - RNA, 20 nt, synthetic construct
  source 1..20: mol_type = other RNA
ggaggctgaagccgcggcgg

SEQ ID NO: 15194 - RNA, 20 nt, synthetic construct
  source 1..20: mol_type = other RNA
ccgccgcggcttcagcctcc

SEQ ID NO: 15195 - RNA, 20 nt, synthetic construct
  source 1..20: mol_type = other RNA
ggctgaagccgcggcggggg

SEQ ID NO: 15196 - RNA, 20 nt, synthetic construct
  source 1..20: mol_type = other RNA
tgaagccgcggcgggggcgg

SEQ ID NO: 15197 - RNA, 20 nt, synthetic construct
  source 1..20: mol_type = other RNA
cgcggcgggggcggcggccg

SEQ ID NO: 15198 - RNA, 20 nt, synthetic construct
  source 1..20: mol_type = other RNA
ctcggccgccgcccccgccg

SEQ ID NO: 15199 - RNA, 20 nt, synthetic construct
  source 1..20: mol_type = other RNA
ggggcggcggccgaggactc

SEQ ID NO: 15200 - RNA, 20 nt, synthetic construct
  source 1..20: mol_type = other RNA
gaggactccggcgccgcacg

SEQ ID NO: 15201 - RNA, 20 nt, synthetic construct
  source 1..20: mol_type = other RNA
tcgtgcggcgccggagtcct

SEQ ID NO: 15202 - RNA, 20 nt, synthetic construct
  source 1..20: mol_type = other RNA
caggctgcctcgtgcggcgc

SEQ ID NO: 15203 - RNA, 20 nt, synthetic construct
  source 1..20: mol_type = other RNA
cgcacgaggcagcctgcagc

SEQ ID NO: 15204 - RNA, 20 nt, synthetic construct
  source 1..20: mol_type = other RNA
cggctgcaggctgcctcgtg

SEQ ID NO: 15205 - RNA, 20 nt, synthetic construct
  source 1..20: mol_type = other RNA
aggcagcctgcagccggccc

SEQ ID NO: 15206 - RNA, 20 nt, synthetic construct
  source 1..20: mol_type = other RNA
gctgggccggggccggctgc

SEQ ID NO: 15207 - RNA, 20 nt, synthetic construct
  source 1..20: mol_type = other RNA
ccggccccggcccagccccc

SEQ ID NO: 15208 - RNA, 20 nt, synthetic construct
  source 1..20: mol_type = other RNA
cggccccggcccagccccct

SEQ ID NO: 15209 - RNA, 20 nt, synthetic construct
  source 1..20: mol_type = other RNA
ggccccggcccagccccctg

SEQ ID NO: 15210 - RNA, 20 nt, synthetic construct
  source 1..20: mol_type = other RNA
ccagggggctgggccggggc

SEQ ID NO: 15211 - RNA, 20 nt, synthetic construct
  source 1..20: mol_type = other RNA
gtccccagggggctgggccg

SEQ ID NO: 15212 - RNA, 20 nt, synthetic construct
  source 1..20: mol_type = other RNA
ggtccccagggggctgggcc

SEQ ID NO: 15213 - RNA, 20 nt, synthetic construct
  source 1..20: mol_type = other RNA
gggtccccagggggctgggc

SEQ ID NO: 15214 - RNA, 20 nt, synthetic construct
  source 1..20: mol_type = other RNA
tgcggggtccccagggggct

SEQ ID NO: 15215 - RNA, 20 nt, synthetic construct
  source 1..20: mol_type = other RNA
ctgcggggtccccagggggc

SEQ ID NO: 15216 - RNA, 20 nt, synthetic construct
  source 1..20: mol_type = other RNA
ccctggggaccccgcagccc

SEQ ID NO: 15217 - RNA, 20 nt, synthetic construct
  source 1..20: mol_type = other RNA
tgggctgcggggtccccagg

SEQ ID NO: 15218 - RNA, 20 nt, synthetic construct
  source 1..20: mol_type = other RNA
ctgggctgcggggtccccag

SEQ ID NO: 15219 - RNA, 20 nt, synthetic construct
  source 1..20: mol_type = other RNA
cctgggctgcggggtcccca

SEQ ID NO: 15220 - RNA, 20 nt, synthetic construct
  source 1..20: mol_type = other RNA
ggaccccgcagcccaggcct

SEQ ID NO: 15221 - RNA, 20 nt, synthetic construct
  source 1..20: mol_type = other RNA
tgaccgaggcctgggctgcg

SEQ ID NO: 15222 - RNA, 20 nt, synthetic construct
  source 1..20: mol_type = other RNA
ctgaccgaggcctgggctgc

SEQ ID NO: 15223 - RNA, 20 nt, synthetic construct
  source 1..20: mol_type = other RNA
gctgaccgaggcctgggctg

SEQ ID NO: 15224 - RNA, 20 nt, synthetic construct
  source 1..20: mol_type = other RNA
gccgttgctgaccgaggcct

SEQ ID NO: 15225 - RNA, 20 nt, synthetic construct
  source 1..20: mol_type = other RNA
cgccgttgctgaccgaggcc

SEQ ID NO: 15226 - RNA, 20 nt, synthetic construct
  source 1..20: mol_type = other RNA
ggtcagcaacggcgaagacg

SEQ ID NO: 15227 - RNA, 20 nt, synthetic construct
  source 1..20: mol_type = other RNA
gtcagcaacggcgaagacgc

SEQ ID NO: 15228 - RNA, 20 nt, synthetic construct
  source 1..20: mol_type = other RNA
agcaacggcgaagacgcggg

SEQ ID NO: 15229 - RNA, 20 nt, synthetic construct
  source 1..20: mol_type = other RNA
aacggcgaagacgcgggcgg

SEQ ID NO: 15230 - RNA, 20 nt, synthetic construct
  source 1..20: mol_type = other RNA
cgaagacgcgggcggcggcg

SEQ ID NO: 15231 - RNA, 20 nt, synthetic construct
  source 1..20: mol_type = other RNA
gaagacgcgggcggcggcgc

SEQ ID NO: 15232 - RNA, 20 nt, synthetic construct
  source 1..20: mol_type = other RNA
acgcgggcggcggcgcgggc

SEQ ID NO: 15233 - RNA, 20 nt, synthetic construct
  source 1..20: mol_type = other RNA
cgcgggcggcggcgcgggca

SEQ ID NO: 15234 - RNA, 20 nt, synthetic construct
  source 1..20: mol_type = other RNA
cggcggcgcgggcagggagc

SEQ ID NO: 15235 - RNA, 20 nt, synthetic construct
  source 1..20: mol_type = other RNA
cggcgcgggcagggagctgg

SEQ ID NO: 15236 - RNA, 20 nt, synthetic construct
  source 1..20: mol_type = other RNA
tggtggacttgaagatcatc

SEQ ID NO: 15237 - RNA, 20 nt, synthetic construct
  source 1..20: mol_type = other RNA
gcatgacgtgaagttccccc

SEQ ID NO: 15238 - RNA, 20 nt, synthetic construct
  source 1..20: mol_type = other RNA
ggggaacttcacgtcatgct

SEQ ID NO: 15239 - RNA, 20 nt, synthetic construct
  source 1..20: mol_type = other RNA
aagttccccctggacagcac

SEQ ID NO: 15240 - RNA, 20 nt, synthetic construct
  source 1..20: mol_type = other RNA
cggagcctgtgctgtccagg

SEQ ID NO: 15241 - RNA, 20 nt, synthetic construct
  source 1..20: mol_type = other RNA
tcggagcctgtgctgtccag

SEQ ID NO: 15242 - RNA, 20 nt, synthetic construct
  source 1..20: mol_type = other RNA
ctcggagcctgtgctgtcca

SEQ ID NO: 15243 - RNA, 20 nt, synthetic construct
  source 1..20: mol_type = other RNA
gctcggagcctgtgctgtcc

SEQ ID NO: 15244 - RNA, 20 nt, synthetic construct
  source 1..20: mol_type = other RNA
gtggatcttctgtttcagct

SEQ ID NO: 15245 - RNA, 20 nt, synthetic construct
  source 1..20: mol_type = other RNA
cagaagatccactcgattac

SEQ ID NO: 15246 - RNA, 20 nt, synthetic construct
  source 1..20: mol_type = other RNA
tcgattacaggtaattcctg

SEQ ID NO: 15247 - RNA, 20 nt, synthetic construct
  source 1..20: mol_type = other RNA
aggaattacctgtaatcgag

SEQ ID NO: 15248 - RNA, 20 nt, synthetic construct
  source 1..20: mol_type = other RNA
agactggctgtcagcgccac

SEQ ID NO: 15249 - RNA, 20 nt, synthetic construct
  source 1..20: mol_type = other RNA
ggaggcggggtggggaagac

SEQ ID NO: 15250 - RNA, 20 nt, synthetic construct
  source 1..20: mol_type = other RNA
ttccccaccccgcctcctga

SEQ ID NO: 15251 - RNA, 20 nt, synthetic construct
  source 1..20: mol_type = other RNA
ggccatcaggaggcggggtg

SEQ ID NO: 15252 - RNA, 20 nt, synthetic construct
  source 1..20: mol_type = other RNA
gggccatcaggaggcggggt

SEQ ID NO: 15253 - RNA, 20 nt, synthetic construct
  source 1..20: mol_type = other RNA
agggccatcaggaggcgggg

SEQ ID NO: 15254 - RNA, 20 nt, synthetic construct
  source 1..20: mol_type = other RNA
gcaagggccatcaggaggcg

SEQ ID NO: 15255 - RNA, 20 nt, synthetic construct
  source 1..20: mol_type = other RNA
tgcaagggccatcaggaggc

SEQ ID NO: 15256 - RNA, 20 nt, synthetic construct
  source 1..20: mol_type = other RNA
gtgcaagggccatcaggagg

SEQ ID NO: 15257 - RNA, 20 nt, synthetic construct
  source 1..20: mol_type = other RNA
agggtgcaagggccatcagg

SEQ ID NO: 15258 - RNA, 20 nt, synthetic construct
  source 1..20: mol_type = other RNA
gatggcccttgcaccctact

SEQ ID NO: 15259 - RNA, 20 nt, synthetic construct
  source 1..20: mol_type = other RNA
agtagggtgcaagggccatc

SEQ ID NO: 15260 - RNA, 20 nt, synthetic construct
  source 1..20: mol_type = other RNA
cttgcaccctactaggcacc

SEQ ID NO: 15261 - RNA, 20 nt, synthetic construct
  source 1..20: mol_type = other RNA
gcaccctactaggcacctgg

SEQ ID NO: 15262 - RNA, 20 nt, synthetic construct
  source 1..20: mol_type = other RNA
caggtgcctagtagggtgca

SEQ ID NO: 15263 - RNA, 20 nt, synthetic construct
  source 1..20: mol_type = other RNA
aagccaccaggtgcctagta

SEQ ID NO: 15264 - RNA, 20 nt, synthetic construct
  source 1..20: mol_type = other RNA
aaagccaccaggtgcctagt

SEQ ID NO: 15265 - RNA, 20 nt, synthetic construct
  source 1..20: mol_type = other RNA
ctggtggctttccttgcatc

SEQ ID NO: 15266 - RNA, 20 nt, synthetic construct
  source 1..20: mol_type = other RNA
ctgatgcaaggaaagccacc

SEQ ID NO: 15267 - RNA, 20 nt, synthetic construct
  source 1..20: mol_type = other RNA
ggatggggggacctgatgca

SEQ ID NO: 15268 - RNA, 20 nt, synthetic construct
  source 1..20: mol_type = other RNA
aagactgctgtaaggatggg

SEQ ID NO: 15269 - RNA, 20 nt, synthetic construct
  source 1..20: mol_type = other RNA
gaagactgctgtaaggatgg

SEQ ID NO: 15270 - RNA, 20 nt, synthetic construct
  source 1..20: mol_type = other RNA
tccttacagcagtcttctga

SEQ ID NO: 15271 - RNA, 20 nt, synthetic construct
  source 1..20: mol_type = other RNA
cagaagactgctgtaaggat

SEQ ID NO: 15272 - RNA, 20 nt, synthetic construct
  source 1..20: mol_type = other RNA
tggaggcagtattcactttt

SEQ ID NO: 15273 - RNA, 20 nt, synthetic construct
  source 1..20: mol_type = other RNA
atggatactacacagctctt

SEQ ID NO: 15274 - RNA, 20 nt, synthetic construct
  source 1..20: mol_type = other RNA
aggaaggacagaaaaatgta

SEQ ID NO: 15275 - RNA, 20 nt, synthetic construct
  source 1..20: mol_type = other RNA
gtggacagtgaaaggaagga

SEQ ID NO: 15276 - RNA, 20 nt, synthetic construct
  source 1..20: mol_type = other RNA
gaaggtggacagtgaaagga

SEQ ID NO: 15277 - RNA, 20 nt, synthetic construct
  source 1..20: mol_type = other RNA
ggtagaaggtggacagtgaa

SEQ ID NO: 15278 - RNA, 20 nt, synthetic construct
  source 1..20: mol_type = other RNA
ccaccttctaccttttccca

SEQ ID NO: 15279 - RNA, 20 nt, synthetic construct
  source 1..20: mol_type = other RNA
ccttgggaaaaggtagaagg

SEQ ID NO: 15280 - RNA, 20 nt, synthetic construct
  source 1..20: mol_type = other RNA
agaccttgggaaaaggtaga

SEQ ID NO: 15281 - RNA, 20 nt, synthetic construct
  source 1..20: mol_type = other RNA
aggcgggagaccttgggaaa

SEQ ID NO: 15282 - RNA, 20 nt, synthetic construct
  source 1..20: mol_type = other RNA
catggcaggcgggagacctt

SEQ ID NO: 15283 - RNA, 20 nt, synthetic construct
  source 1..20: mol_type = other RNA
gcatggcaggcgggagacct

SEQ ID NO: 15284 - RNA, 20 nt, synthetic construct
  source 1..20: mol_type = other RNA
tgactttctgcatggcaggc

SEQ ID NO: 15285 - RNA, 20 nt, synthetic construct
  source 1..20: mol_type = other RNA
atgactttctgcatggcagg

SEQ ID NO: 15286 - RNA, 20 nt, synthetic construct
  source 1..20: mol_type = other RNA
catgcagaaagtcatgtata

SEQ ID NO: 15287 - RNA, 20 nt, synthetic construct
  source 1..20: mol_type = other RNA
atgcagaaagtcatgtataa

SEQ ID NO: 15288 - RNA, 20 nt, synthetic construct
  source 1..20: mol_type = other RNA
cttatacatgactttctgca

SEQ ID NO: 15289 - RNA, 20 nt, synthetic construct
  source 1..20: mol_type = other RNA
gtataagggactcgtccccg

SEQ ID NO: 15290 - RNA, 20 nt, synthetic construct
  source 1..20: mol_type = other RNA
ctctcaatgttttatcctcg

SEQ ID NO: 15291 - RNA, 20 nt, synthetic construct
  source 1..20: mol_type = other RNA
tctctcaatgttttatcctc

SEQ ID NO: 15292 - RNA, 20 nt, synthetic construct
  source 1..20: mol_type = other RNA
ttctctcaatgttttatcct

SEQ ID NO: 15293 - RNA, 20 nt, synthetic construct
  source 1..20: mol_type = other RNA
agagaaataaaagtgaccag

SEQ ID NO: 15294 - RNA, 20 nt, synthetic construct
  source 1..20: mol_type = other RNA
gagaaataaaagtgaccagt

SEQ ID NO: 15295 - RNA, 20 nt, synthetic construct
  source 1..20: mol_type = other RNA
agaaataaaagtgaccagtg

SEQ ID NO: 15296 - RNA, 20 nt, synthetic construct
  source 1..20: mol_type = other RNA
gaccagtggggccaagatca

SEQ ID NO: 15297 - RNA, 20 nt, synthetic construct
  source 1..20: mol_type = other RNA
cagtggggccaagatcatgg

SEQ ID NO: 15298 - RNA, 20 nt, synthetic construct
  source 1..20: mol_type = other RNA
ggggccaagatcatggtggt

SEQ ID NO: 15299 - RNA, 20 nt, synthetic construct
  source 1..20: mol_type = other RNA
ggagccaaccaccatgatct

SEQ ID NO: 15300 - RNA, 20 nt, synthetic construct
  source 1..20: mol_type = other RNA
tgctaaaacatcattgatgg

SEQ ID NO: 15301 - RNA, 20 nt, synthetic construct
  source 1..20: mol_type = other RNA
tactgctaaaacatcattga

SEQ ID NO: 15302 - RNA, 20 nt, synthetic construct
  source 1..20: mol_type = other RNA
acccaaagatgctgcgcagc

SEQ ID NO: 15303 - RNA, 20 nt, synthetic construct
  source 1..20: mol_type = other RNA
tcctgctgcgcagcatcttt

SEQ ID NO: 15304 - RNA, 20 nt, synthetic construct
  source 1..20: mol_type = other RNA
atcctgctgcgcagcatctt

SEQ ID NO: 15305 - RNA, 20 nt, synthetic construct
  source 1..20: mol_type = other RNA
tgctgcgcagcaggatgcaa

SEQ ID NO: 15306 - RNA, 20 nt, synthetic construct
  source 1..20: mol_type = other RNA
aaaggccgaagagaacaaga

SEQ ID NO: 15307 - RNA, 20 nt, synthetic construct
  source 1..20: mol_type = other RNA
aggctccttcttgttctctt

SEQ ID NO: 15308 - RNA, 20 nt, synthetic construct
  source 1..20: mol_type = other RNA
acaagaaggagcctctctgc

SEQ ID NO: 15309 - RNA, 20 nt, synthetic construct
  source 1..20: mol_type = other RNA
ctcactttctgcctgcagag

SEQ ID NO: 15310 - RNA, 20 nt, synthetic construct
  source 1..20: mol_type = other RNA
tgagtccatcttgtgcttct

SEQ ID NO: 15311 - RNA, 20 nt, synthetic construct
  source 1..20: mol_type = other RNA
caagaccaagaagcacaaga

SEQ ID NO: 15312 - RNA, 20 nt, synthetic construct
  source 1..20: mol_type = other RNA
tcttggtcttgagaaatttg

SEQ ID NO: 15313 - RNA, 20 nt, synthetic construct
  source 1..20: mol_type = other RNA
ggctttgtcctcttgagccg

SEQ ID NO: 15314 - RNA, 20 nt, synthetic construct
  source 1..20: mol_type = other RNA
ttgtcctcttgagccgtggc

SEQ ID NO: 15315 - RNA, 20 nt, synthetic construct
  source 1..20: mol_type = other RNA
ataaccagccacggctcaag

SEQ ID NO: 15316 - RNA, 20 nt, synthetic construct
  source 1..20: mol_type = other RNA
agggagaatataaccagcca

SEQ ID NO: 15317 - RNA, 20 nt, synthetic construct
  source 1..20: mol_type = other RNA
ccctagaataagctcctttt

SEQ ID NO: 15318 - RNA, 20 nt, synthetic construct
  source 1..20: mol_type = other RNA
gaataagctcctttttggac

SEQ ID NO: 15319 - RNA, 20 nt, synthetic construct
  source 1..20: mol_type = other RNA
aataagctcctttttggaca

SEQ ID NO: 15320 - RNA, 20 nt, synthetic construct
  source 1..20: mol_type = other RNA
tttttggacagggcccatga

SEQ ID NO: 15321 - RNA, 20 nt, synthetic construct
  source 1..20: mol_type = other RNA
atcatgggccctgtccaaaa

SEQ ID NO: 15322 - RNA, 20 nt, synthetic construct
  source 1..20: mol_type = other RNA
gggcccatgatggaaattta

SEQ ID NO: 15323 - RNA, 20 nt, synthetic construct
  source 1..20: mol_type = other RNA
ctgccataaatttccatcat

SEQ ID NO: 15324 - RNA, 20 nt, synthetic construct
  source 1..20: mol_type = other RNA
gctgccataaatttccatca

SEQ ID NO: 15325 - RNA, 20 nt, synthetic construct
  source 1..20: mol_type = other RNA
tggaaatttatggcagcagt

SEQ ID NO: 15326 - RNA, 20 nt, synthetic construct
  source 1..20: mol_type = other RNA
ggaaatttatggcagcagtt

SEQ ID NO: 15327 - RNA, 20 nt, synthetic construct
  source 1..20: mol_type = other RNA
agcagttgggtgccgcagag

SEQ ID NO: 15328 - RNA, 20 nt, synthetic construct
  source 1..20: mol_type = other RNA
agttgggtgccgcagagtgg

SEQ ID NO: 15329 - RNA, 20 nt, synthetic construct
  source 1..20: mol_type = other RNA
tagttgtcacctccactctg

SEQ ID NO: 15330 - RNA, 20 nt, synthetic construct
  source 1..20: mol_type = other RNA
gagacaaagttgcaaatctc

SEQ ID NO: 15331 - RNA, 20 nt, synthetic construct
  source 1..20: mol_type = other RNA
atttgcaactttgtctcatc

SEQ ID NO: 15332 - RNA, 20 nt, synthetic construct
  source 1..20: mol_type = other RNA
tgcaactttgtctcatctgg

SEQ ID NO: 15333 - RNA, 20 nt, synthetic construct
  source 1..20: mol_type = other RNA
gcaactttgtctcatctggc

SEQ ID NO: 15334 - RNA, 20 nt, synthetic construct
  source 1..20: mol_type = other RNA
gtctcaagtctacctacttt

SEQ ID NO: 15335 - RNA, 20 nt, synthetic construct
  source 1..20: mol_type = other RNA
cctactttaggataagacct

SEQ ID NO: 15336 - RNA, 20 nt, synthetic construct
  source 1..20: mol_type = other RNA
ccaaggtcttatcctaaagt

SEQ ID NO: 15337 - RNA, 20 nt, synthetic construct
  source 1..20: mol_type = other RNA
ttaggataagaccttggtaa

SEQ ID NO: 15338 - RNA, 20 nt, synthetic construct
  source 1..20: mol_type = other RNA
taggataagaccttggtaaa

SEQ ID NO: 15339 - RNA, 20 nt, synthetic construct
  source 1..20: mol_type = other RNA
gataagaccttggtaaaggg

SEQ ID NO: 15340 - RNA, 20 nt, synthetic construct
  source 1..20: mol_type = other RNA
tctgaagcctccctttacca

SEQ ID NO: 15341 - RNA, 20 nt, synthetic construct
  source 1..20: mol_type = other RNA
gcttcagaccatgtgttgaa

SEQ ID NO: 15342 - RNA, 20 nt, synthetic construct
  source 1..20: mol_type = other RNA
gtgttgaaaggaatcagacg

SEQ ID NO: 15343 - RNA, 20 nt, synthetic construct
  source 1..20: mol_type = other RNA
tgttgaaaggaatcagacgt

SEQ ID NO: 15344 - RNA, 20 nt, synthetic construct
  source 1..20: mol_type = other RNA
gcttttgagccaaaacacta

SEQ ID NO: 15345 - RNA, 20 nt, synthetic construct
  source 1..20: mol_type = other RNA
tgaagaaagccttagtgttt

SEQ ID NO: 15346 - RNA, 20 nt, synthetic construct
  source 1..20: mol_type = other RNA
tttcttcatcctctctttca

SEQ ID NO: 15347 - RNA, 20 nt, synthetic construct
  source 1..20: mol_type = other RNA
ttcttcatcctctctttcaa

SEQ ID NO: 15348 - RNA, 20 nt, synthetic construct
  source 1..20: mol_type = other RNA
ttactattcccttgaaagag

SEQ ID NO: 15349 - RNA, 20 nt, synthetic construct
  source 1..20: mol_type = other RNA
cttctgacttatagcaacac

SEQ ID NO: 15350 - RNA, 20 nt, synthetic construct
  source 1..20: mol_type = other RNA
atagcaacacaggaaagtgt

SEQ ID NO: 15351 - RNA, 20 nt, synthetic construct
  source 1..20: mol_type = other RNA
cacaggaaagtgttggataa

SEQ ID NO: 15352 - RNA, 20 nt, synthetic construct
  source 1..20: mol_type = other RNA
acagatggcatcacatcttc

SEQ ID NO: 15353 - RNA, 20 nt, synthetic construct
  source 1..20: mol_type = other RNA
gatgtgatgccatctgttaa

SEQ ID NO: 15354 - RNA, 20 nt, synthetic construct
  source 1..20: mol_type = other RNA
atgtgatgccatctgttaag

SEQ ID NO: 15355 - RNA, 20 nt, synthetic construct
  source 1..20: mol_type = other RNA
tgtgatgccatctgttaagg

SEQ ID NO: 15356 - RNA, 20 nt, synthetic construct
  source 1..20: mol_type = other RNA
gccatctgttaagggggccc

SEQ ID NO: 15357 - RNA, 20 nt, synthetic construct
  source 1..20: mol_type = other RNA
ctgttaagggggcccaggta

SEQ ID NO: 15358 - RNA, 20 nt, synthetic construct
  source 1..20: mol_type = other RNA
acctgggcccccttaacaga

SEQ ID NO: 15359 - RNA, 20 nt, synthetic construct
  source 1..20: mol_type = other RNA
ttaagggggcccaggtaagg

SEQ ID NO: 15360 - RNA, 20 nt, synthetic construct
  source 1..20: mol_type = other RNA
caaagaaatccgccttacct

SEQ ID NO: 15361 - RNA, 20 nt, synthetic construct
  source 1..20: mol_type = other RNA
acaaagaaatccgccttacc

SEQ ID NO: 15362 - RNA, 20 nt, synthetic construct
  source 1..20: mol_type = other RNA
ttgtgagcattctgaaaatg

SEQ ID NO: 15363 - RNA, 20 nt, synthetic construct
  source 1..20: mol_type = other RNA
cagccccaccgtctgacttg

SEQ ID NO: 15364 - RNA, 20 nt, synthetic construct
  source 1..20: mol_type = other RNA
gaacctcaagtcagacggtg

SEQ ID NO: 15365 - RNA, 20 nt, synthetic construct
  source 1..20: mol_type = other RNA
ggaacctcaagtcagacggt

SEQ ID NO: 15366 - RNA, 20 nt, synthetic construct
  source 1..20: mol_type = other RNA
aggaacctcaagtcagacgg

SEQ ID NO: 15367 - RNA, 20 nt, synthetic construct
  source 1..20: mol_type = other RNA
tggaggaacctcaagtcaga

SEQ ID NO: 15368 - RNA, 20 nt, synthetic construct
  source 1..20: mol_type = other RNA
aagagaagggacaggattgg

SEQ ID NO: 15369 - RNA, 20 nt, synthetic construct
  source 1..20: mol_type = other RNA
aaaaagagaagggacaggat

SEQ ID NO: 15370 - RNA, 20 nt, synthetic construct
  source 1..20: mol_type = other RNA
agggaaaaaagagaagggac

SEQ ID NO: 15371 - RNA, 20 nt, synthetic construct
  source 1..20: mol_type = other RNA
aaaacagggaaaaaagagaa

SEQ ID NO: 15372 - RNA, 20 nt, synthetic construct
  source 1..20: mol_type = other RNA
aaaaacagggaaaaaagaga

SEQ ID NO: 15373 - RNA, 20 nt, synthetic construct
  source 1..20: mol_type = other RNA
gtctcaaaaaaaaaaaaaca

SEQ ID NO: 15374 - RNA, 20 nt, synthetic construct
  source 1..20: mol_type = other RNA
tgtctcaaaaaaaaaaaaac

SEQ ID NO: 15375 - RNA, 20 nt, synthetic construct
  source 1..20: mol_type = other RNA
caaagcggtcagatcacctg

SEQ ID NO: 15376 - RNA, 20 nt, synthetic construct
  source 1..20: mol_type = other RNA
gctttggcctcccagtgtgc

SEQ ID NO: 15377 - RNA, 20 nt, synthetic construct
  source 1..20: mol_type = other RNA
ctttggcctcccagtgtgct

SEQ ID NO: 15378 - RNA, 20 nt, synthetic construct
  source 1..20: mol_type = other RNA
agcacactgggaggccaaag

SEQ ID NO: 15379 - RNA, 20 nt, synthetic construct
  source 1..20: mol_type = other RNA
tcccagtgtgctgggattac

SEQ ID NO: 15380 - RNA, 20 nt, synthetic construct
  source 1..20: mol_type = other RNA
tgtaatcccagcacactggg

SEQ ID NO: 15381 - RNA, 20 nt, synthetic construct
  source 1..20: mol_type = other RNA
gcctgtaatcccagcacact

SEQ ID NO: 15382 - RNA, 20 nt, synthetic construct
  source 1..20: mol_type = other RNA
cgcctgtaatcccagcacac

SEQ ID NO: 15383 - RNA, 20 nt, synthetic construct
  source 1..20: mol_type = other RNA
caggcgtgagccaccgcgct

SEQ ID NO: 15384 - RNA, 20 nt, synthetic construct
  source 1..20: mol_type = other RNA
gagaagggggccaagcgcgg

SEQ ID NO: 15385 - RNA, 20 nt, synthetic construct
  source 1..20: mol_type = other RNA
aaagagaagggggccaagcg

SEQ ID NO: 15386 - RNA, 20 nt, synthetic construct
  source 1..20: mol_type = other RNA
agtcagaaaaaaagagaagg

SEQ ID NO: 15387 - RNA, 20 nt, synthetic construct
  source 1..20: mol_type = other RNA
cagtcagaaaaaaagagaag

SEQ ID NO: 15388 - RNA, 20 nt, synthetic construct
  source 1..20: mol_type = other RNA
acagtcagaaaaaaagagaa

SEQ ID NO: 15389 - RNA, 20 nt, synthetic construct
  source 1..20: mol_type = other RNA
gacagtcagaaaaaaagaga

SEQ ID NO: 15390 - RNA, 20 nt, synthetic construct
  source 1..20: mol_type = other RNA
agagaatggtaagagatgga

SEQ ID NO: 15391 - RNA, 20 nt, synthetic construct
  source 1..20: mol_type = other RNA
gagagaatggtaagagatgg

SEQ ID NO: 15392 - RNA, 20 nt, synthetic construct
  source 1..20: mol_type = other RNA
cacgagagaatggtaagaga

SEQ ID NO: 15393 - RNA, 20 nt, synthetic construct
  source 1..20: mol_type = other RNA
taccattctctcgtgccttc

SEQ ID NO: 15394 - RNA, 20 nt, synthetic construct
  source 1..20: mol_type = other RNA
ctcctgaaggcacgagagaa

SEQ ID NO: 15395 - RNA, 20 nt, synthetic construct
  source 1..20: mol_type = other RNA
ccttcaggagcgcctgccaa

SEQ ID NO: 15396 - RNA, 20 nt, synthetic construct
  source 1..20: mol_type = other RNA
ccgttggcaggcgctcctga

SEQ ID NO: 15397 - RNA, 20 nt, synthetic construct
  source 1..20: mol_type = other RNA
ctgccaacggtaccgctgtc

SEQ ID NO: 15398 - RNA, 20 nt, synthetic construct
  source 1..20: mol_type = other RNA
cggacagcggtaccgttggc

SEQ ID NO: 15399 - RNA, 20 nt, synthetic construct
  source 1..20: mol_type = other RNA
atgccggacagcggtaccgt

SEQ ID NO: 15400 - RNA, 20 nt, synthetic construct
  source 1..20: mol_type = other RNA
ttattgtacatgccggacag

SEQ ID NO: 15401 - RNA, 20 nt, synthetic construct
  source 1..20: mol_type = other RNA
tccggcatgtacaataaatc

SEQ ID NO: 15402 - RNA, 20 nt, synthetic construct
  source 1..20: mol_type = other RNA
ggcatgtacaataaatctgg

SEQ ID NO: 15403 - RNA, 20 nt, synthetic construct
  source 1..20: mol_type = other RNA
tccagatttattgtacatgc

SEQ ID NO: 15404 - RNA, 20 nt, synthetic construct
  source 1..20: mol_type = other RNA
ctggtcttgttctagtttaa

SEQ ID NO: 15405 - RNA, 20 nt, synthetic construct
  source 1..20: mol_type = other RNA
aactagaacaagaccagctg

SEQ ID NO: 15406 - RNA, 20 nt, synthetic construct
  source 1..20: mol_type = other RNA
gaacaagaccagctgtggat

SEQ ID NO: 15407 - RNA, 20 nt, synthetic construct
  source 1..20: mol_type = other RNA
cagctgtggattggcactaa

SEQ ID NO: 15408 - RNA, 20 nt, synthetic construct
  source 1..20: mol_type = other RNA
ctttagtgccaatccacagc

SEQ ID NO: 15409 - RNA, 20 nt, synthetic construct
  source 1..20: mol_type = other RNA
gttcttcctcgcctccttgc

SEQ ID NO: 15410 - RNA, 20 nt, synthetic construct
  source 1..20: mol_type = other RNA
agtgggccagcaaggaggcg

SEQ ID NO: 15411 - RNA, 20 nt, synthetic construct
  source 1..20: mol_type = other RNA
caggcagtgggccagcaagg

SEQ ID NO: 15412 - RNA, 20 nt, synthetic construct
  source 1..20: mol_type = other RNA
gctggcccactgcctgcctc

SEQ ID NO: 15413 - RNA, 20 nt, synthetic construct
  source 1..20: mol_type = other RNA
aggcaggcagtgggccagca

SEQ ID NO: 15414 - RNA, 20 nt, synthetic construct
  source 1..20: mol_type = other RNA
gggtgccagaggcaggcagt

SEQ ID NO: 15415 - RNA, 20 nt, synthetic construct
  source 1..20: mol_type = other RNA
tgggtgccagaggcaggcag

SEQ ID NO: 15416 - RNA, 20 nt, synthetic construct
  source 1..20: mol_type = other RNA
tgctgctgggtgccagaggc

SEQ ID NO: 15417 - RNA, 20 nt, synthetic construct
  source 1..20: mol_type = other RNA
tgagtgctgctgggtgccag

SEQ ID NO: 15418 - RNA, 20 nt, synthetic construct
  source 1..20: mol_type = other RNA
tctaaaatgtgagtgctgct

SEQ ID NO: 15419 - RNA, 20 nt, synthetic construct
  source 1..20: mol_type = other RNA
ctctaaaatgtgagtgctgc

SEQ ID NO: 15420 - RNA, 20 nt, synthetic construct
  source 1..20: mol_type = other RNA
gagagaggtttcagaaggag

SEQ ID NO: 15421 - RNA, 20 nt, synthetic construct
  source 1..20: mol_type = other RNA
agagagaggtttcagaagga

SEQ ID NO: 15422 - RNA, 20 nt, synthetic construct
  source 1..20: mol_type = other RNA
gagagagaggtttcagaagg

SEQ ID NO: 15423 - RNA, 20 nt, synthetic construct
  source 1..20: mol_type = other RNA
gtggagagagaggtttcaga

SEQ ID NO: 15424 - RNA, 20 nt, synthetic construct
  source 1..20: mol_type = other RNA
gcaaagcacagtggagagag

SEQ ID NO: 15425 - RNA, 20 nt, synthetic construct
  source 1..20: mol_type = other RNA
ggtggggggagaatcaagga

SEQ ID NO: 15426 - RNA, 20 nt, synthetic construct
  source 1..20: mol_type = other RNA
ggagggtggggggagaatca

SEQ ID NO: 15427 - RNA, 20 nt, synthetic construct
  source 1..20: mol_type = other RNA
caagtcatttggagggtggg

SEQ ID NO: 15428 - RNA, 20 nt, synthetic construct
  source 1..20: mol_type = other RNA
gcaagtcatttggagggtgg

SEQ ID NO: 15429 - RNA, 20 nt, synthetic construct
  source 1..20: mol_type = other RNA
agcaagtcatttggagggtg

SEQ ID NO: 15430 - RNA, 20 nt, synthetic construct
  source 1..20: mol_type = other RNA
cagcaagtcatttggagggt

SEQ ID NO: 15431 - RNA, 20 nt, synthetic construct
  source 1..20: mol_type = other RNA
gcagcaagtcatttggaggg

SEQ ID NO: 15432 - RNA, 20 nt, synthetic construct
  source 1..20: mol_type = other RNA
gcggcagcaagtcatttgga

SEQ ID NO: 15433 - RNA, 20 nt, synthetic construct
  source 1..20: mol_type = other RNA
agcggcagcaagtcatttgg

SEQ ID NO: 15434 - RNA, 20 nt, synthetic construct
  source 1..20: mol_type = other RNA
agaagcggcagcaagtcatt

SEQ ID NO: 15435 - RNA, 20 nt, synthetic construct
  source 1..20: mol_type = other RNA
aagcgctctatgaacagaag

SEQ ID NO: 15436 - RNA, 20 nt, synthetic construct
  source 1..20: mol_type = other RNA
agagagtaatgagtgctctg

SEQ ID NO: 15437 - RNA, 20 nt, synthetic construct
  source 1..20: mol_type = other RNA
cagagagtaatgagtgctct

SEQ ID NO: 15438 - RNA, 20 nt, synthetic construct
  source 1..20: mol_type = other RNA
tcagagagtaatgagtgctc

SEQ ID NO: 15439 - RNA, 20 nt, synthetic construct
  source 1..20: mol_type = other RNA
ctgtccccctgttagattcc

SEQ ID NO: 15440 - RNA, 20 nt, synthetic construct
  source 1..20: mol_type = other RNA
tccccctgttagattcctgg

SEQ ID NO: 15441 - RNA, 20 nt, synthetic construct
  source 1..20: mol_type = other RNA
ccccctgttagattcctgga

SEQ ID NO: 15442 - RNA, 20 nt, synthetic construct
  source 1..20: mol_type = other RNA
ccctccaggaatctaacagg

SEQ ID NO: 15443 - RNA, 20 nt, synthetic construct
  source 1..20: mol_type = other RNA
tccctccaggaatctaacag

SEQ ID NO: 15444 - RNA, 20 nt, synthetic construct
  source 1..20: mol_type = other RNA
ttccctccaggaatctaaca

SEQ ID NO: 15445 - RNA, 20 nt, synthetic construct
  source 1..20: mol_type = other RNA
gttccctccaggaatctaac

SEQ ID NO: 15446 - RNA, 20 nt, synthetic construct
  source 1..20: mol_type = other RNA
aggcatgttcggttccctcc

SEQ ID NO: 15447 - RNA, 20 nt, synthetic construct
  source 1..20: mol_type = other RNA
acaggtgatttaggcatgtt

SEQ ID NO: 15448 - RNA, 20 nt, synthetic construct
  source 1..20: mol_type = other RNA
tggtcagaaacaggtgattt

SEQ ID NO: 15449 - RNA, 20 nt, synthetic construct
  source 1..20: mol_type = other RNA
ctgtttctgaccagcactgt

SEQ ID NO: 15450 - RNA, 20 nt, synthetic construct
  source 1..20: mol_type = other RNA
ctacagtgctggtcagaaac

SEQ ID NO: 15451 - RNA, 20 nt, synthetic construct
  source 1..20: mol_type = other RNA
acactgaatacctacagtgc

SEQ ID NO: 15452 - RNA, 20 nt, synthetic construct
  source 1..20: mol_type = other RNA
ctgtaggtattcagtgttcg

SEQ ID NO: 15453 - RNA, 20 nt, synthetic construct
  source 1..20: mol_type = other RNA
taaatgctaaagagaagtat

SEQ ID NO: 15454 - RNA, 20 nt, synthetic construct
  source 1..20: mol_type = other RNA
aaatgctaaagagaagtata

SEQ ID NO: 15455 - RNA, 20 nt, synthetic construct
  source 1..20: mol_type = other RNA
aatgctaaagagaagtatag

SEQ ID NO: 15456 - RNA, 20 nt, synthetic construct
  source 1..20: mol_type = other RNA
atgctaaagagaagtatagg

SEQ ID NO: 15457 - RNA, 20 nt, synthetic construct
  source 1..20: mol_type = other RNA
tcccatcatctgacgttcac

SEQ ID NO: 15458 - RNA, 20 nt, synthetic construct
  source 1..20: mol_type = other RNA
accagtgaacgtcagatgat

SEQ ID NO: 15459 - RNA, 20 nt, synthetic construct
  source 1..20: mol_type = other RNA
aaccagtgaacgtcagatga

SEQ ID NO: 15460 - RNA, 20 nt, synthetic construct
  source 1..20: mol_type = other RNA
tctgacgttcactggtttca

SEQ ID NO: 15461 - RNA, 20 nt, synthetic construct
  source 1..20: mol_type = other RNA
tagtgagactccacttaaaa

SEQ ID NO: 15462 - RNA, 20 nt, synthetic construct
  source 1..20: mol_type = other RNA
agtgagactccacttaaaat

SEQ ID NO: 15463 - RNA, 20 nt, synthetic construct
  source 1..20: mol_type = other RNA
taaaatgggaccaagtttta

SEQ ID NO: 15464 - RNA, 20 nt, synthetic construct
  source 1..20: mol_type = other RNA
caagttttatggagaataat

SEQ ID NO: 15465 - RNA, 20 nt, synthetic construct
  source 1..20: mol_type = other RNA
aagttttatggagaataatt

SEQ ID NO: 15466 - RNA, 20 nt, synthetic construct
  source 1..20: mol_type = other RNA
agttttatggagaataattg

SEQ ID NO: 15467 - RNA, 20 nt, synthetic construct
  source 1..20: mol_type = other RNA
caattattctccataaaact

SEQ ID NO: 15468 - RNA, 20 nt, synthetic construct
  source 1..20: mol_type = other RNA
ttatggagaataattggggc

SEQ ID NO: 15469 - RNA, 20 nt, synthetic construct
  source 1..20: mol_type = other RNA
tatggagaataattggggca

SEQ ID NO: 15470 - RNA, 20 nt, synthetic construct
  source 1..20: mol_type = other RNA
atggagaataattggggcag

SEQ ID NO: 15471 - RNA, 20 nt, synthetic construct
  source 1..20: mol_type = other RNA
ggttccccccagtttttgca

SEQ ID NO: 15472 - RNA, 20 nt, synthetic construct
  source 1..20: mol_type = other RNA
gttccccccagtttttgcaa

SEQ ID NO: 15473 - RNA, 20 nt, synthetic construct
  source 1..20: mol_type = other RNA
aggcccttgcaaaaactggg

SEQ ID NO: 15474 - RNA, 20 nt, synthetic construct
  source 1..20: mol_type = other RNA
aaggcccttgcaaaaactgg

SEQ ID NO: 15475 - RNA, 20 nt, synthetic construct
  source 1..20: mol_type = other RNA
aaaggcccttgcaaaaactg

SEQ ID NO: 15476 - RNA, 20 nt, synthetic construct
  source 1..20: mol_type = other RNA
caaaggcccttgcaaaaact

SEQ ID NO: 15477 - RNA, 20 nt, synthetic construct
  source 1..20: mol_type = other RNA
tcaaaggcccttgcaaaaac

SEQ ID NO: 15478 - RNA, 20 nt, synthetic construct
  source 1..20: mol_type = other RNA
tgatctagcagagggttcaa

SEQ ID NO: 15479 - RNA, 20 nt, synthetic construct
  source 1..20: mol_type = other RNA
gaagagaatgatctagcaga

SEQ ID NO: 15480 - RNA, 20 nt, synthetic construct
  source 1..20: mol_type = other RNA
agaagagaatgatctagcag

SEQ ID NO: 15481 - RNA, 20 nt, synthetic construct
  source 1..20: mol_type = other RNA
ctgataaagggaagatggac

SEQ ID NO: 15482 - RNA, 20 nt, synthetic construct
  source 1..20: mol_type = other RNA
tactactgataaagggaaga

SEQ ID NO: 15483 - RNA, 20 nt, synthetic construct
  source 1..20: mol_type = other RNA
ggcagcttactactgataaa

SEQ ID NO: 15484 - RNA, 20 nt, synthetic construct
  source 1..20: mol_type = other RNA
gggcagcttactactgataa

SEQ ID NO: 15485 - RNA, 20 nt, synthetic construct
  source 1..20: mol_type = other RNA
ccagcctctgtcaactttgc

SEQ ID NO: 15486 - RNA, 20 nt, synthetic construct
  source 1..20: mol_type = other RNA
ctgcaaagttgacagaggct

SEQ ID NO: 15487 - RNA, 20 nt, synthetic construct
  source 1..20: mol_type = other RNA
cctgcaaagttgacagaggc

SEQ ID NO: 15488 - RNA, 20 nt, synthetic construct
  source 1..20: mol_type = other RNA
atcacctgcaaagttgacag

SEQ ID NO: 15489 - RNA, 20 nt, synthetic construct
  source 1..20: mol_type = other RNA
atagacttcctgcctcttgc

SEQ ID NO: 15490 - RNA, 20 nt, synthetic construct
  source 1..20: mol_type = other RNA
gtagaggtccagcaagaggc

SEQ ID NO: 15491 - RNA, 20 nt, synthetic construct
  source 1..20: mol_type = other RNA
aaaagtagaggtccagcaag

SEQ ID NO: 15492 - RNA, 20 nt, synthetic construct
  source 1..20: mol_type = other RNA
tggacctctacttttgcttg

SEQ ID NO: 15493 - RNA, 20 nt, synthetic construct
  source 1..20: mol_type = other RNA
ggacctctacttttgcttgt

SEQ ID NO: 15494 - RNA, 20 nt, synthetic construct
  source 1..20: mol_type = other RNA
ctgcccacaagcaaaagtag

SEQ ID NO: 15495 - RNA, 20 nt, synthetic construct
  source 1..20: mol_type = other RNA
cttgtgggcagcctcattga

SEQ ID NO: 15496 - RNA, 20 nt, synthetic construct
  source 1..20: mol_type = other RNA
ctcattgaaggcagttgcta

SEQ ID NO: 15497 - RNA, 20 nt, synthetic construct
  source 1..20: mol_type = other RNA
cgtagcaactgccttcaatg

SEQ ID NO: 15498 - RNA, 20 nt, synthetic construct
  source 1..20: mol_type = other RNA
ggcagttgctacggctgacc

SEQ ID NO: 15499 - RNA, 20 nt, synthetic construct
  source 1..20: mol_type = other RNA
cttcatggcagggtctttcc

SEQ ID NO: 15500 - RNA, 20 nt, synthetic construct
  source 1..20: mol_type = other RNA
cctgccatgaagataggtgc

SEQ ID NO: 15501 - RNA, 20 nt, synthetic construct
  source 1..20: mol_type = other RNA
ctgcacctatcttcatggca

SEQ ID NO: 15502 - RNA, 20 nt, synthetic construct
  source 1..20: mol_type = other RNA
cctgcacctatcttcatggc

SEQ ID NO: 15503 - RNA, 20 nt, synthetic construct
  source 1..20: mol_type = other RNA
tctgcctgcacctatcttca

SEQ ID NO: 15504 - RNA, 20 nt, synthetic construct
  source 1..20: mol_type = other RNA
taggtgcaggcagagaagtc

SEQ ID NO: 15505 - RNA, 20 nt, synthetic construct
  source 1..20: mol_type = other RNA
tgcaggcagagaagtctgga

SEQ ID NO: 15506 - RNA, 20 nt, synthetic construct
  source 1..20: mol_type = other RNA
gcaggcagagaagtctggat

SEQ ID NO: 15507 - RNA, 20 nt, synthetic construct
  source 1..20: mol_type = other RNA
ctaagtctgtaagtgctcat

SEQ ID NO: 15508 - RNA, 20 nt, synthetic construct
  source 1..20: mol_type = other RNA
gtaagtgctcattggttcct

SEQ ID NO: 15509 - RNA, 20 nt, synthetic construct
  source 1..20: mol_type = other RNA
taagtgctcattggttcctt

SEQ ID NO: 15510 - RNA, 20 nt, synthetic construct
  source 1..20: mol_type = other RNA
aagtgctcattggttccttg

SEQ ID NO: 15511 - RNA, 20 nt, synthetic construct
  source 1..20: mol_type = other RNA
ttggggaatatttctgtgtc

SEQ ID NO: 15512 - RNA, 20 nt, synthetic construct
  source 1..20: mol_type = other RNA
tgacacagaaatattcccca

SEQ ID NO: 15513 - RNA, 20 nt, synthetic construct
  source 1..20: mol_type = other RNA
tctgtgtcaggaagttgtat

SEQ ID NO: 15514 - RNA, 20 nt, synthetic construct
  source 1..20: mol_type = other RNA
ctgtgtcaggaagttgtata

SEQ ID NO: 15515 - RNA, 20 nt, synthetic construct
  source 1..20: mol_type = other RNA
agggaacacatcataactgc

SEQ ID NO: 15516 - RNA, 20 nt, synthetic construct
  source 1..20: mol_type = other RNA
agaacttcctgaccctgtat

SEQ ID NO: 15517 - RNA, 20 nt, synthetic construct
  source 1..20: mol_type = other RNA
aaaacttccaatacagggtc

SEQ ID NO: 15518 - RNA, 20 nt, synthetic construct
  source 1..20: mol_type = other RNA
aaaagaaaacttccaataca

SEQ ID NO: 15519 - RNA, 20 nt, synthetic construct
  source 1..20: mol_type = other RNA
aaaaagaaaacttccaatac

SEQ ID NO: 15520 - RNA, 20 nt, synthetic construct
  source 1..20: mol_type = other RNA
gaagttttctttttgctagt

SEQ ID NO: 15521 - RNA, 20 nt, synthetic construct
  source 1..20: mol_type = other RNA
gagcagccgccttcctgctt

SEQ ID NO: 15522 - RNA, 20 nt, synthetic construct
  source 1..20: mol_type = other RNA
gccttcctgctttggcctaa

SEQ ID NO: 15523 - RNA, 20 nt, synthetic construct
  source 1..20: mol_type = other RNA
ccttcctgctttggcctaaa

SEQ ID NO: 15524 - RNA, 20 nt, synthetic construct
  source 1..20: mol_type = other RNA
tttaggccaaagcaggaagg

SEQ ID NO: 15525 - RNA, 20 nt, synthetic construct
  source 1..20: mol_type = other RNA
ccctttaggccaaagcagga

SEQ ID NO: 15526 - RNA, 20 nt, synthetic construct
  source 1..20: mol_type = other RNA
ctctccctttaggccaaagc

SEQ ID NO: 15527 - RNA, 20 nt, synthetic construct
  source 1..20: mol_type = other RNA
tcttctacagctctcccttt

SEQ ID NO: 15528 - RNA, 20 nt, synthetic construct
  source 1..20: mol_type = other RNA
gtagaagaagctcaatatgt

SEQ ID NO: 15529 - RNA, 20 nt, synthetic construct
  source 1..20: mol_type = other RNA
tagaagaagctcaatatgtt

SEQ ID NO: 15530 - RNA, 20 nt, synthetic construct
  source 1..20: mol_type = other RNA
agaagaagctcaatatgttg

SEQ ID NO: 15531 - RNA, 20 nt, synthetic construct
  source 1..20: mol_type = other RNA
gtgagtaaggaggctttcaa

SEQ ID NO: 15532 - RNA, 20 nt, synthetic construct
  source 1..20: mol_type = other RNA
ggtgagtaaggaggctttca

SEQ ID NO: 15533 - RNA, 20 nt, synthetic construct
  source 1..20: mol_type = other RNA
cttactcaccagtcttgttg

SEQ ID NO: 15534 - RNA, 20 nt, synthetic construct
  source 1..20: mol_type = other RNA
aacaagactggtgagtaagg

SEQ ID NO: 15535 - RNA, 20 nt, synthetic construct
  source 1..20: mol_type = other RNA
ctcaacaagactggtgagta

SEQ ID NO: 15536 - RNA, 20 nt, synthetic construct
  source 1..20: mol_type = other RNA
accagtcttgttgaggagca

SEQ ID NO: 15537 - RNA, 20 nt, synthetic construct
  source 1..20: mol_type = other RNA
gccatgctcctcaacaagac

SEQ ID NO: 15538 - RNA, 20 nt, synthetic construct
  source 1..20: mol_type = other RNA
atggactactcatgttttct

SEQ ID NO: 15539 - RNA, 20 nt, synthetic construct
  source 1..20: mol_type = other RNA
tggactactcatgttttcta

SEQ ID NO: 15540 - RNA, 20 nt, synthetic construct
  source 1..20: mol_type = other RNA
tagaaaacatgagtagtcca

SEQ ID NO: 15541 - RNA, 20 nt, synthetic construct
  source 1..20: mol_type = other RNA
atgttttctagggttgaaca

SEQ ID NO: 15542 - RNA, 20 nt, synthetic construct
  source 1..20: mol_type = other RNA
cacccatagcactgtacctc

SEQ ID NO: 15543 - RNA, 20 nt, synthetic construct
  source 1..20: mol_type = other RNA
agaggtacagtgctatgggt

SEQ ID NO: 15544 - RNA, 20 nt, synthetic construct
  source 1..20: mol_type = other RNA
cagaggtacagtgctatggg

SEQ ID NO: 15545 - RNA, 20 nt, synthetic construct
  source 1..20: mol_type = other RNA
ctccagaggtacagtgctat

SEQ ID NO: 15546 - RNA, 20 nt, synthetic construct
  source 1..20: mol_type = other RNA
gctccagaggtacagtgcta

SEQ ID NO: 15547 - RNA, 20 nt, synthetic construct
  source 1..20: mol_type = other RNA
cactgtacctctggagccca

SEQ ID NO: 15548 - RNA, 20 nt, synthetic construct
  source 1..20: mol_type = other RNA
actgtacctctggagcccaa

SEQ ID NO: 15549 - RNA, 20 nt, synthetic construct
  source 1..20: mol_type = other RNA
ctgtacctctggagcccaag

SEQ ID NO: 15550 - RNA, 20 nt, synthetic construct
  source 1..20: mol_type = other RNA
acctctggagcccaaggggc

SEQ ID NO: 15551 - RNA, 20 nt, synthetic construct
  source 1..20: mol_type = other RNA
gcctgccccttgggctccag

SEQ ID NO: 15552 - RNA, 20 nt, synthetic construct
  source 1..20: mol_type = other RNA
gacaagactgcctgcccctt

SEQ ID NO: 15553 - RNA, 20 nt, synthetic construct
  source 1..20: mol_type = other RNA
tgacaagactgcctgcccct

SEQ ID NO: 15554 - RNA, 20 nt, synthetic construct
  source 1..20: mol_type = other RNA
gacacttaggtaacaggact

SEQ ID NO: 15555 - RNA, 20 nt, synthetic construct
  source 1..20: mol_type = other RNA
tgacacttaggtaacaggac

SEQ ID NO: 15556 - RNA, 20 nt, synthetic construct
  source 1..20: mol_type = other RNA
gcttatgacacttaggtaac

SEQ ID NO: 15557 - RNA, 20 nt, synthetic construct
  source 1..20: mol_type = other RNA
tatgagtgcttatgacactt

SEQ ID NO: 15558 - RNA, 20 nt, synthetic construct
  source 1..20: mol_type = other RNA
cataagaggacagcttgttc

SEQ ID NO: 15559 - RNA, 20 nt, synthetic construct
  source 1..20: mol_type = other RNA
ataagaggacagcttgttct

SEQ ID NO: 15560 - RNA, 20 nt, synthetic construct
  source 1..20: mol_type = other RNA
ggacagcttgttctgggagt

SEQ ID NO: 15561 - RNA, 20 nt, synthetic construct
  source 1..20: mol_type = other RNA
gggagttggctgctagccac

SEQ ID NO: 15562 - RNA, 20 nt, synthetic construct
  source 1..20: mol_type = other RNA
cactggcttcgtctttctgc

SEQ ID NO: 15563 - RNA, 20 nt, synthetic construct
  source 1..20: mol_type = other RNA
cagcagaaagacgaagccag

SEQ ID NO: 15564 - RNA, 20 nt, synthetic construct
  source 1..20: mol_type = other RNA
tttctgctggcaagaagaag

SEQ ID NO: 15565 - RNA, 20 nt, synthetic construct
  source 1..20: mol_type = other RNA
ctggcaagaagaagcggcta

SEQ ID NO: 15566 - RNA, 20 nt, synthetic construct
  source 1..20: mol_type = other RNA
tgaccatcccagcagcgagt

SEQ ID NO: 15567 - RNA, 20 nt, synthetic construct
  source 1..20: mol_type = other RNA
aggccaactcgctgctggga

SEQ ID NO: 15568 - RNA, 20 nt, synthetic construct
  source 1..20: mol_type = other RNA
gcagcgagttggcctcttcg

SEQ ID NO: 15569 - RNA, 20 nt, synthetic construct
  source 1..20: mol_type = other RNA
gaagaggccaactcgctgct

SEQ ID NO: 15570 - RNA, 20 nt, synthetic construct
  source 1..20: mol_type = other RNA
agcgagttggcctcttcgtg

SEQ ID NO: 15571 - RNA, 20 nt, synthetic construct
  source 1..20: mol_type = other RNA
cagcaaagcgccccacgaag

SEQ ID NO: 15572 - RNA, 20 nt, synthetic construct
  source 1..20: mol_type = other RNA
tgctgagtaagtgaccctta

SEQ ID NO: 15573 - RNA, 20 nt, synthetic construct
  source 1..20: mol_type = other RNA
gctgagtaagtgacccttaa

SEQ ID NO: 15574 - RNA, 20 nt, synthetic construct
  source 1..20: mol_type = other RNA
tcaagagtagcagcccttaa

SEQ ID NO: 15575 - RNA, 20 nt, synthetic construct
  source 1..20: mol_type = other RNA
gtcaagagtagcagccctta

SEQ ID NO: 15576 - RNA, 20 nt, synthetic construct
  source 1..20: mol_type = other RNA
taaactctgctagcttgtgt

SEQ ID NO: 15577 - RNA, 20 nt, synthetic construct
  source 1..20: mol_type = other RNA
actctgctagcttgtgtagg

SEQ ID NO: 15578 - RNA, 20 nt, synthetic construct
  source 1..20: mol_type = other RNA
ctgctagcttgtgtaggagg

SEQ ID NO: 15579 - RNA, 20 nt, synthetic construct
  source 1..20: mol_type = other RNA
agcttgttctcattcttttg

SEQ ID NO: 15580 - RNA, 20 nt, synthetic construct
  source 1..20: mol_type = other RNA
aatgagaacaagctccaggc

SEQ ID NO: 15581 - RNA, 20 nt, synthetic construct
  source 1..20: mol_type = other RNA
acaagctccaggcaggaaac

SEQ ID NO: 15582 - RNA, 20 nt, synthetic construct
  source 1..20: mol_type = other RNA
ggcaggaaaccggaagccgc

SEQ ID NO: 15583 - RNA, 20 nt, synthetic construct
  source 1..20: mol_type = other RNA
gcggcttccggtttcctgcc

SEQ ID NO: 15584 - RNA, 20 nt, synthetic construct
  source 1..20: mol_type = other RNA
aggaaaccggaagccgctgg

SEQ ID NO: 15585 - RNA, 20 nt, synthetic construct
  source 1..20: mol_type = other RNA
tgctctcctccagcggcttc

SEQ ID NO: 15586 - RNA, 20 nt, synthetic construct
  source 1..20: mol_type = other RNA
gggtacatgctctcctccag

SEQ ID NO: 15587 - RNA, 20 nt, synthetic construct
  source 1..20: mol_type = other RNA
agagcatgtaccctgctcgt

SEQ ID NO: 15588 - RNA, 20 nt, synthetic construct
  source 1..20: mol_type = other RNA
gctcgtaggaaagttgaatc

SEQ ID NO: 15589 - RNA, 20 nt, synthetic construct
  source 1..20: mol_type = other RNA
attcaactttcctacgagca

SEQ ID NO: 15590 - RNA, 20 nt, synthetic construct
  source 1..20: mol_type = other RNA
gattcaactttcctacgagc

SEQ ID NO: 15591 - RNA, 20 nt, synthetic construct
  source 1..20: mol_type = other RNA
ggaaagttgaatctggctga

SEQ ID NO: 15592 - RNA, 20 nt, synthetic construct
  source 1..20: mol_type = other RNA
gaaggtctgatgtagtgatc

SEQ ID NO: 15593 - RNA, 20 nt, synthetic construct
  source 1..20: mol_type = other RNA
tgatgtagtgatcaggagtg

SEQ ID NO: 15594 - RNA, 20 nt, synthetic construct
  source 1..20: mol_type = other RNA
gatgtagtgatcaggagtgt

SEQ ID NO: 15595 - RNA, 20 nt, synthetic construct
  source 1..20: mol_type = other RNA
gtccagaattgcccaatttt

SEQ ID NO: 15596 - RNA, 20 nt, synthetic construct
  source 1..20: mol_type = other RNA
ctccaaaaattgggcaattc

SEQ ID NO: 15597 - RNA, 20 nt, synthetic construct
  source 1..20: mol_type = other RNA
tcttgaaaactccaaaaatt

SEQ ID NO: 15598 - RNA, 20 nt, synthetic construct
  source 1..20: mol_type = other RNA
ctcttgaaaactccaaaaat

SEQ ID NO: 15599 - RNA, 20 nt, synthetic construct
  source 1..20: mol_type = other RNA
aaaaatatacaacagatttc

SEQ ID NO: 15600 - RNA, 20 nt, synthetic construct
  source 1..20: mol_type = other RNA
gtgaaatctccagacatttc

SEQ ID NO: 15601 - RNA, 20 nt, synthetic construct
  source 1..20: mol_type = other RNA
tccagacatttcaggatgaa

SEQ ID NO: 15602 - RNA, 20 nt, synthetic construct
  source 1..20: mol_type = other RNA
acctttcatcctgaaatgtc

SEQ ID NO: 15603 - RNA, 20 nt, synthetic construct
  source 1..20: mol_type = other RNA
cttaaagacagctgctgccc

SEQ ID NO: 15604 - RNA, 20 nt, synthetic construct
  source 1..20: mol_type = other RNA
ggcagcagctgtctttaaga

SEQ ID NO: 15605 - RNA, 20 nt, synthetic construct
  source 1..20: mol_type = other RNA
tgctgcccaggtcctgcttt

SEQ ID NO: 15606 - RNA, 20 nt, synthetic construct
  source 1..20: mol_type = other RNA
gctgcccaggtcctgcttta

SEQ ID NO: 15607 - RNA, 20 nt, synthetic construct
  source 1..20: mol_type = other RNA
tcggccctaaagcaggacct

SEQ ID NO: 15608 - RNA, 20 nt, synthetic construct
  source 1..20: mol_type = other RNA
gtcggccctaaagcaggacc

SEQ ID NO: 15609 - RNA, 20 nt, synthetic construct
  source 1..20: mol_type = other RNA
acaacagtcggccctaaagc

SEQ ID NO: 15610 - RNA, 20 nt, synthetic construct
  source 1..20: mol_type = other RNA
tctagtggctctacaacagt

SEQ ID NO: 15611 - RNA, 20 nt, synthetic construct
  source 1..20: mol_type = other RNA
atttaggtttggacttctag

SEQ ID NO: 15612 - RNA, 20 nt, synthetic construct
  source 1..20: mol_type = other RNA
aaacctaaataaacatcttc

SEQ ID NO: 15613 - RNA, 20 nt, synthetic construct
  source 1..20: mol_type = other RNA
tgaagatgtttatttaggtt

SEQ ID NO: 15614 - RNA, 20 nt, synthetic construct
  source 1..20: mol_type = other RNA
ggacctgaagatgtttattt

SEQ ID NO: 15615 - RNA, 20 nt, synthetic construct
  source 1..20: mol_type = other RNA
aaaatgggggctggggagaa

SEQ ID NO: 15616 - RNA, 20 nt, synthetic construct
  source 1..20: mol_type = other RNA
aaaaatgggggctggggaga

SEQ ID NO: 15617 - RNA, 20 nt, synthetic construct
  source 1..20: mol_type = other RNA
tatctgaaaaatgggggctg

SEQ ID NO: 15618 - RNA, 20 nt, synthetic construct
  source 1..20: mol_type = other RNA
cccccatttttcagatactg

SEQ ID NO: 15619 - RNA, 20 nt, synthetic construct
  source 1..20: mol_type = other RNA
agtatctgaaaaatgggggc

SEQ ID NO: 15620 - RNA, 20 nt, synthetic construct
  source 1..20: mol_type = other RNA
cctcagtatctgaaaaatgg

SEQ ID NO: 15621 - RNA, 20 nt, synthetic construct
  source 1..20: mol_type = other RNA
gcctcagtatctgaaaaatg

SEQ ID NO: 15622 - RNA, 20 nt, synthetic construct
  source 1..20: mol_type = other RNA
ggcctcagtatctgaaaaat

SEQ ID NO: 15623 - RNA, 20 nt, synthetic construct
  source 1..20: mol_type = other RNA
gggcctcagtatctgaaaaa

SEQ ID NO: 15624 - RNA, 20 nt, synthetic construct
  source 1..20: mol_type = other RNA
acattttacttcagttctgt

SEQ ID NO: 15625 - RNA, 20 nt, synthetic construct
  source 1..20: mol_type = other RNA
gacattttacttcagttctg

SEQ ID NO: 15626 - RNA, 20 nt, synthetic construct
  source 1..20: mol_type = other RNA
ccccagctagaccagaacgc

SEQ ID NO: 15627 - RNA, 20 nt, synthetic construct
  source 1..20: mol_type = other RNA
ccagcgttctggtctagctg

SEQ ID NO: 15628 - RNA, 20 nt, synthetic construct
  source 1..20: mol_type = other RNA
accagcgttctggtctagct

SEQ ID NO: 15629 - RNA, 20 nt, synthetic construct
  source 1..20: mol_type = other RNA
gaccagcgttctggtctagc

SEQ ID NO: 15630 - RNA, 20 nt, synthetic construct
  source 1..20: mol_type = other RNA
gaatttagagaccagcgttc

SEQ ID NO: 15631 - RNA, 20 nt, synthetic construct
  source 1..20: mol_type = other RNA
ctctaaattcctagtctgtt

SEQ ID NO: 15632 - RNA, 20 nt, synthetic construct
  source 1..20: mol_type = other RNA
ataagttggccaaacagact

SEQ ID NO: 15633 - RNA, 20 nt, synthetic construct
  source 1..20: mol_type = other RNA
gagtctaaaaatagataagt

SEQ ID NO: 15634 - RNA, 20 nt, synthetic construct
  source 1..20: mol_type = other RNA
ccagatttttctttctgcaa

SEQ ID NO: 15635 - RNA, 20 nt, synthetic construct
  source 1..20: mol_type = other RNA
cctttgcagaaagaaaaatc

SEQ ID NO: 15636 - RNA, 20 nt, synthetic construct
  source 1..20: mol_type = other RNA
gctgcaagtttttttccact

SEQ ID NO: 15637 - RNA, 20 nt, synthetic construct
  source 1..20: mol_type = other RNA
cagcaaacagctaaaccaag

SEQ ID NO: 15638 - RNA, 20 nt, synthetic construct
  source 1..20: mol_type = other RNA
gcagggggaggggggcaggg

SEQ ID NO: 15639 - RNA, 20 nt, synthetic construct
  source 1..20: mol_type = other RNA
ggcgcagggggaggggggca

SEQ ID NO: 15640 - RNA, 20 nt, synthetic construct
  source 1..20: mol_type = other RNA
gggcgcagggggaggggggc

SEQ ID NO: 15641 - RNA, 20 nt, synthetic construct
  source 1..20: mol_type = other RNA
acgggggcgcagggggaggg

SEQ ID NO: 15642 - RNA, 20 nt, synthetic construct
  source 1..20: mol_type = other RNA
gacgggggcgcagggggagg

SEQ ID NO: 15643 - RNA, 20 nt, synthetic construct
  source 1..20: mol_type = other RNA
ggacgggggcgcagggggag

SEQ ID NO: 15644 - RNA, 20 nt, synthetic construct
  source 1..20: mol_type = other RNA
gggacgggggcgcaggggga

SEQ ID NO: 15645 - RNA, 20 nt, synthetic construct
  source 1..20: mol_type = other RNA
agggacgggggcgcaggggg

SEQ ID NO: 15646 - RNA, 20 nt, synthetic construct
  source 1..20: mol_type = other RNA
ctcagggacgggggcgcagg

SEQ ID NO: 15647 - RNA, 20 nt, synthetic construct
  source 1..20: mol_type = other RNA
cctcagggacgggggcgcag

SEQ ID NO: 15648 - RNA, 20 nt, synthetic construct
  source 1..20: mol_type = other RNA
acctcagggacgggggcgca

SEQ ID NO: 15649 - RNA, 20 nt, synthetic construct
  source 1..20: mol_type = other RNA
cacctcagggacgggggcgc

SEQ ID NO: 15650 - RNA, 20 nt, synthetic construct
  source 1..20: mol_type = other RNA
agcagacacctcagggacgg

SEQ ID NO: 15651 - RNA, 20 nt, synthetic construct
  source 1..20: mol_type = other RNA
cagcagacacctcagggacg

SEQ ID NO: 15652 - RNA, 20 nt, synthetic construct
  source 1..20: mol_type = other RNA
gcagcagacacctcagggac

SEQ ID NO: 15653 - RNA, 20 nt, synthetic construct
  source 1..20: mol_type = other RNA
agcagcagacacctcaggga

SEQ ID NO: 15654 - RNA, 20 nt, synthetic construct
  source 1..20: mol_type = other RNA
ctggagcagcagacacctca

SEQ ID NO: 15655 - RNA, 20 nt, synthetic construct
  source 1..20: mol_type = other RNA
cctggagcagcagacacctc

SEQ ID NO: 15656 - RNA, 20 nt, synthetic construct
  source 1..20: mol_type = other RNA
atggccatgtccccttgtgc

SEQ ID NO: 15657 - RNA, 20 nt, synthetic construct
  source 1..20: mol_type = other RNA
tgcacctgcacaaggggaca

SEQ ID NO: 15658 - RNA, 20 nt, synthetic construct
  source 1..20: mol_type = other RNA
gcgaggtgcacctgcacaag

SEQ ID NO: 15659 - RNA, 20 nt, synthetic construct
  source 1..20: mol_type = other RNA
ggcgaggtgcacctgcacaa

SEQ ID NO: 15660 - RNA, 20 nt, synthetic construct
  source 1..20: mol_type = other RNA
aggcgaggtgcacctgcaca

SEQ ID NO: 15661 - RNA, 20 nt, synthetic construct
  source 1..20: mol_type = other RNA
gggtgaggtcaggggaggcg

SEQ ID NO: 15662 - RNA, 20 nt, synthetic construct
  source 1..20: mol_type = other RNA
ggactgggtgaggtcagggg

SEQ ID NO: 15663 - RNA, 20 nt, synthetic construct
  source 1..20: mol_type = other RNA
gcgggactgggtgaggtcag

SEQ ID NO: 15664 - RNA, 20 nt, synthetic construct
  source 1..20: mol_type = other RNA
agcgggactgggtgaggtca

SEQ ID NO: 15665 - RNA, 20 nt, synthetic construct
  source 1..20: mol_type = other RNA
aagcgggactgggtgaggtc

SEQ ID NO: 15666 - RNA, 20 nt, synthetic construct
  source 1..20: mol_type = other RNA
tcacccagtcccgcttcact

SEQ ID NO: 15667 - RNA, 20 nt, synthetic construct
  source 1..20: mol_type = other RNA
aagtgaagcgggactgggtg

SEQ ID NO: 15668 - RNA, 20 nt, synthetic construct
  source 1..20: mol_type = other RNA
gagccaagtgaagcgggact

SEQ ID NO: 15669 - RNA, 20 nt, synthetic construct
  source 1..20: mol_type = other RNA
tgagccaagtgaagcgggac

SEQ ID NO: 15670 - RNA, 20 nt, synthetic construct
  source 1..20: mol_type = other RNA
cgcttcacttggctcactcc

SEQ ID NO: 15671 - RNA, 20 nt, synthetic construct
  source 1..20: mol_type = other RNA
gggagtgagccaagtgaagc

SEQ ID NO: 15672 - RNA, 20 nt, synthetic construct
  source 1..20: mol_type = other RNA
cgggagtgagccaagtgaag

SEQ ID NO: 15673 - RNA, 20 nt, synthetic construct
  source 1..20: mol_type = other RNA
cggcagtctcatctcactcc

SEQ ID NO: 15674 - RNA, 20 nt, synthetic construct
  source 1..20: mol_type = other RNA
tggagtgagatgagactgcc

SEQ ID NO: 15675 - RNA, 20 nt, synthetic construct
  source 1..20: mol_type = other RNA
ctggagtgagatgagactgc

SEQ ID NO: 15676 - RNA, 20 nt, synthetic construct
  source 1..20: mol_type = other RNA
agggggcagcaagggatgcc

SEQ ID NO: 15677 - RNA, 20 nt, synthetic construct
  source 1..20: mol_type = other RNA
gtaagagaagggggcagcaa

SEQ ID NO: 15678 - RNA, 20 nt, synthetic construct
  source 1..20: mol_type = other RNA
ggtaagagaagggggcagca

SEQ ID NO: 15679 - RNA, 20 nt, synthetic construct
  source 1..20: mol_type = other RNA
ggatggcaggtaagagaagg

SEQ ID NO: 15680 - RNA, 20 nt, synthetic construct
  source 1..20: mol_type = other RNA
aggatggcaggtaagagaag

SEQ ID NO: 15681 - RNA, 20 nt, synthetic construct
  source 1..20: mol_type = other RNA
gaggatggcaggtaagagaa

SEQ ID NO: 15682 - RNA, 20 nt, synthetic construct
  source 1..20: mol_type = other RNA
ggaggatggcaggtaagaga

SEQ ID NO: 15683 - RNA, 20 nt, synthetic construct
  source 1..20: mol_type = other RNA
gcgagtttaaggaggatggc

SEQ ID NO: 15684 - RNA, 20 nt, synthetic construct
  source 1..20: mol_type = other RNA
tgaggcgagtttaaggagga

SEQ ID NO: 15685 - RNA, 20 nt, synthetic construct
  source 1..20: mol_type = other RNA
acattgaggcgagtttaagg

SEQ ID NO: 15686 - RNA, 20 nt, synthetic construct
  source 1..20: mol_type = other RNA
aagacattgaggcgagttta

SEQ ID NO: 15687 - RNA, 20 nt, synthetic construct
  source 1..20: mol_type = other RNA
catggggtcagaagacattg

SEQ ID NO: 15688 - RNA, 20 nt, synthetic construct
  source 1..20: mol_type = other RNA
ttctgaccccatgtgatcag

SEQ ID NO: 15689 - RNA, 20 nt, synthetic construct
  source 1..20: mol_type = other RNA
gagataccactgatcacatg

SEQ ID NO: 15690 - RNA, 20 nt, synthetic construct
  source 1..20: mol_type = other RNA
tgagataccactgatcacat

SEQ ID NO: 15691 - RNA, 20 nt, synthetic construct
  source 1..20: mol_type = other RNA
ttgagataccactgatcaca

SEQ ID NO: 15692 - RNA, 20 nt, synthetic construct
  source 1..20: mol_type = other RNA
tctcaagtgttaatcacaaa

SEQ ID NO: 15693 - RNA, 20 nt, synthetic construct
  source 1..20: mol_type = other RNA
aagtgtgtgaatatagagtg

SEQ ID NO: 15694 - RNA, 20 nt, synthetic construct
  source 1..20: mol_type = other RNA
tgtgtgaatatagagtgcgg

SEQ ID NO: 15695 - RNA, 20 nt, synthetic construct
  source 1..20: mol_type = other RNA
tatagagtgcggaggactcg

SEQ ID NO: 15696 - RNA, 20 nt, synthetic construct
  source 1..20: mol_type = other RNA
agagtgcggaggactcgagg

SEQ ID NO: 15697 - RNA, 20 nt, synthetic construct
  source 1..20: mol_type = other RNA
gagtgcggaggactcgagga

SEQ ID NO: 15698 - RNA, 20 nt, synthetic construct
  source 1..20: mol_type = other RNA
tgcggaggactcgaggaggg

SEQ ID NO: 15699 - RNA, 20 nt, synthetic construct
  source 1..20: mol_type = other RNA
gaggactcgaggagggaggc

SEQ ID NO: 15700 - RNA, 20 nt, synthetic construct
  source 1..20: mol_type = other RNA
aggactcgaggagggaggcc

SEQ ID NO: 15701 - RNA, 20 nt, synthetic construct
  source 1..20: mol_type = other RNA
ggactcgaggagggaggccg

SEQ ID NO: 15702 - RNA, 20 nt, synthetic construct
  source 1..20: mol_type = other RNA
tcgaggagggaggccgggga

SEQ ID NO: 15703 - RNA, 20 nt, synthetic construct
  source 1..20: mol_type = other RNA
cgaggagggaggccggggaa

SEQ ID NO: 15704 - RNA, 20 nt, synthetic construct
  source 1..20: mol_type = other RNA
gggaggccggggaagggagc

SEQ ID NO: 15705 - RNA, 20 nt, synthetic construct
  source 1..20: mol_type = other RNA
ggaggccggggaagggagca

SEQ ID NO: 15706 - RNA, 20 nt, synthetic construct
  source 1..20: mol_type = other RNA
cggggaagggagcagggtcg

SEQ ID NO: 15707 - RNA, 20 nt, synthetic construct
  source 1..20: mol_type = other RNA
cacgaccctgctcccttccc

SEQ ID NO: 15708 - RNA, 20 nt, synthetic construct
  source 1..20: mol_type = other RNA
agaatctagccctaaaatcc

SEQ ID NO: 15709 - RNA, 20 nt, synthetic construct
  source 1..20: mol_type = other RNA
aggggagtgcctggatttta

SEQ ID NO: 15710 - RNA, 20 nt, synthetic construct
  source 1..20: mol_type = other RNA
aaggggagtgcctggatttt

SEQ ID NO: 15711 - RNA, 20 nt, synthetic construct
  source 1..20: mol_type = other RNA
cacaagggaaggggagtgcc

SEQ ID NO: 15712 - RNA, 20 nt, synthetic construct
  source 1..20: mol_type = other RNA
ccttcccttgtgagagccac

SEQ ID NO: 15713 - RNA, 20 nt, synthetic construct
  source 1..20: mol_type = other RNA
cttcccttgtgagagccaca

SEQ ID NO: 15714 - RNA, 20 nt, synthetic construct
  source 1..20: mol_type = other RNA
ttcccttgtgagagccacag

SEQ ID NO: 15715 - RNA, 20 nt, synthetic construct
  source 1..20: mol_type = other RNA
tgtggctctcacaagggaag

SEQ ID NO: 15716 - RNA, 20 nt, synthetic construct
  source 1..20: mol_type = other RNA
ctgtggctctcacaagggaa

SEQ ID NO: 15717 - RNA, 20 nt, synthetic construct
  source 1..20: mol_type = other RNA
cctgtggctctcacaaggga

SEQ ID NO: 15718 - RNA, 20 nt, synthetic construct
  source 1..20: mol_type = other RNA
ttcccctgtggctctcacaa

SEQ ID NO: 15719 - RNA, 20 nt, synthetic construct
  source 1..20: mol_type = other RNA
gttcccctgtggctctcaca

SEQ ID NO: 15720 - RNA, 20 nt, synthetic construct
  source 1..20: mol_type = other RNA
agaggcaacacgttcccctg

SEQ ID NO: 15721 - RNA, 20 nt, synthetic construct
  source 1..20: mol_type = other RNA
cgtgttgcctctttgttcgt

SEQ ID NO: 15722 - RNA, 20 nt, synthetic construct
  source 1..20: mol_type = other RNA
caagaggcctacgaacaaag

SEQ ID NO: 15723 - RNA, 20 nt, synthetic construct
  source 1..20: mol_type = other RNA
gggcagtagggagagtcaag

SEQ ID NO: 15724 - RNA, 20 nt, synthetic construct
  source 1..20: mol_type = other RNA
gactaaggtcttgggcagta

SEQ ID NO: 15725 - RNA, 20 nt, synthetic construct
  source 1..20: mol_type = other RNA
tgactaaggtcttgggcagt

SEQ ID NO: 15726 - RNA, 20 nt, synthetic construct
  source 1..20: mol_type = other RNA
cccaagaccttagtcaatgc

SEQ ID NO: 15727 - RNA, 20 nt, synthetic construct
  source 1..20: mol_type = other RNA
ccaagaccttagtcaatgct

SEQ ID NO: 15728 - RNA, 20 nt, synthetic construct
  source 1..20: mol_type = other RNA
ccagcattgactaaggtctt

SEQ ID NO: 15729 - RNA, 20 nt, synthetic construct
  source 1..20: mol_type = other RNA
cccagcattgactaaggtct

SEQ ID NO: 15730 - RNA, 20 nt, synthetic construct
  source 1..20: mol_type = other RNA
tgcaagcccagcattgacta

SEQ ID NO: 15731 - RNA, 20 nt, synthetic construct
  source 1..20: mol_type = other RNA
gggcttgcataaggttacaa

SEQ ID NO: 15732 - RNA, 20 nt, synthetic construct
  source 1..20: mol_type = other RNA
aaggttacaaaggaatttct

SEQ ID NO: 15733 - RNA, 20 nt, synthetic construct
  source 1..20: mol_type = other RNA
aggttacaaaggaatttctt

SEQ ID NO: 15734 - RNA, 20 nt, synthetic construct
  source 1..20: mol_type = other RNA
tatatttttttttgttgaga

SEQ ID NO: 15735 - RNA, 20 nt, synthetic construct
  source 1..20: mol_type = other RNA
tgagatggagtttcgctctt

SEQ ID NO: 15736 - RNA, 20 nt, synthetic construct
  source 1..20: mol_type = other RNA
ggagtttcgctctttggccc

SEQ ID NO: 15737 - RNA, 20 nt, synthetic construct
  source 1..20: mol_type = other RNA
tggcccaggctgaagtaaag

SEQ ID NO: 15738 - RNA, 20 nt, synthetic construct
  source 1..20: mol_type = other RNA
atgccactttacttcagcct

SEQ ID NO: 15739 - RNA, 20 nt, synthetic construct
  source 1..20: mol_type = other RNA
catgccactttacttcagcc

SEQ ID NO: 15740 - RNA, 20 nt, synthetic construct
  source 1..20: mol_type = other RNA
gaagtaaagtggcatgatct

SEQ ID NO: 15741 - RNA, 20 nt, synthetic construct
  source 1..20: mol_type = other RNA
tcactgcaacttctgccccc

SEQ ID NO: 15742 - RNA, 20 nt, synthetic construct
  source 1..20: mol_type = other RNA
cactgcaacttctgcccccc

SEQ ID NO: 15743 - RNA, 20 nt, synthetic construct
  source 1..20: mol_type = other RNA
gagaatcgcttgaacccggg

SEQ ID NO: 15744 - RNA, 20 nt, synthetic construct
  source 1..20: mol_type = other RNA
cgagaatcgcttgaacccgg

SEQ ID NO: 15745 - RNA, 20 nt, synthetic construct
  source 1..20: mol_type = other RNA
acgagaatcgcttgaacccg

SEQ ID NO: 15746 - RNA, 20 nt, synthetic construct
  source 1..20: mol_type = other RNA
cacgagaatcgcttgaaccc

SEQ ID NO: 15747 - RNA, 20 nt, synthetic construct
  source 1..20: mol_type = other RNA
gcacgagaatcgcttgaacc

SEQ ID NO: 15748 - RNA, 20 nt, synthetic construct
  source 1..20: mol_type = other RNA
gcttcagcctcctgagtagc

SEQ ID NO: 15749 - RNA, 20 nt, synthetic construct
  source 1..20: mol_type = other RNA
cttcagcctcctgagtagct

SEQ ID NO: 15750 - RNA, 20 nt, synthetic construct
  source 1..20: mol_type = other RNA
tcctgagtagctgggattat

SEQ ID NO: 15751 - RNA, 20 nt, synthetic construct
  source 1..20: mol_type = other RNA
tataatcccagctactcagg

SEQ ID NO: 15752 - RNA, 20 nt, synthetic construct
  source 1..20: mol_type = other RNA
acctataatcccagctactc

SEQ ID NO: 15753 - RNA, 20 nt, synthetic construct
  source 1..20: mol_type = other RNA
taggtgcccaccaccacgcc

SEQ ID NO: 15754 - RNA, 20 nt, synthetic construct
  source 1..20: mol_type = other RNA
aattagccaggcgtggtggt

SEQ ID NO: 15755 - RNA, 20 nt, synthetic construct
  source 1..20: mol_type = other RNA
aaattagccaggcgtggtgg

SEQ ID NO: 15756 - RNA, 20 nt, synthetic construct
  source 1..20: mol_type = other RNA
aaaaaattagccaggcgtgg

SEQ ID NO: 15757 - RNA, 20 nt, synthetic construct
  source 1..20: mol_type = other RNA
tacaaaaaattagccaggcg

SEQ ID NO: 15758 - RNA, 20 nt, synthetic construct
  source 1..20: mol_type = other RNA
aaaaatacaaaaaattagcc

SEQ ID NO: 15759 - RNA, 20 nt, synthetic construct
  source 1..20: mol_type = other RNA
ttttgtatttttagtagaga

SEQ ID NO: 15760 - RNA, 20 nt, synthetic construct
  source 1..20: mol_type = other RNA
tttgtatttttagtagagac

SEQ ID NO: 15761 - RNA, 20 nt, synthetic construct
  source 1..20: mol_type = other RNA
ttgtatttttagtagagacg

SEQ ID NO: 15762 - RNA, 20 nt, synthetic construct
  source 1..20: mol_type = other RNA
gagacggggtttcaccatgc

SEQ ID NO: 15763 - RNA, 20 nt, synthetic construct
  source 1..20: mol_type = other RNA
ggggtttcaccatgctggcc

SEQ ID NO: 15764 - RNA, 20 nt, synthetic construct
  source 1..20: mol_type = other RNA
tttcaccatgctggccaggc

SEQ ID NO: 15765 - RNA, 20 nt, synthetic construct
  source 1..20: mol_type = other RNA
cgagaccagcctggccagca

SEQ ID NO: 15766 - RNA, 20 nt, synthetic construct
  source 1..20: mol_type = other RNA
tcaggagttcgagaccagcc

SEQ ID NO: 15767 - RNA, 20 nt, synthetic construct
  source 1..20: mol_type = other RNA
ggtctcgaactcctgatctc

SEQ ID NO: 15768 - RNA, 20 nt, synthetic construct
  source 1..20: mol_type = other RNA
tgggtggatcacctgagatc

SEQ ID NO: 15769 - RNA, 20 nt, synthetic construct
  source 1..20: mol_type = other RNA
ctcaggtgatccacccacct

SEQ ID NO: 15770 - RNA, 20 nt, synthetic construct
  source 1..20: mol_type = other RNA
caggatttggccaaggtggg

SEQ ID NO: 15771 - RNA, 20 nt, synthetic construct
  source 1..20: mol_type = other RNA
agtcaggatttggccaaggt

SEQ ID NO: 15772 - RNA, 20 nt, synthetic construct
  source 1..20: mol_type = other RNA
gagtcaggatttggccaagg

SEQ ID NO: 15773 - RNA, 20 nt, synthetic construct
  source 1..20: mol_type = other RNA
tgtgagtcaggatttggcca

SEQ ID NO: 15774 - RNA, 20 nt, synthetic construct
  source 1..20: mol_type = other RNA
atcctgactcacaagatgtt

SEQ ID NO: 15775 - RNA, 20 nt, synthetic construct
  source 1..20: mol_type = other RNA
acatcttgtgagtcaggatt

SEQ ID NO: 15776 - RNA, 20 nt, synthetic construct
  source 1..20: mol_type = other RNA
atcctaacatcttgtgagtc

SEQ ID NO: 15777 - RNA, 20 nt, synthetic construct
  source 1..20: mol_type = other RNA
tcacaagatgttaggattac

SEQ ID NO: 15778 - RNA, 20 nt, synthetic construct
  source 1..20: mol_type = other RNA
caggcttgagccaccgcgcc

SEQ ID NO: 15779 - RNA, 20 nt, synthetic construct
  source 1..20: mol_type = other RNA
ccaccgcgcctggcctttct

SEQ ID NO: 15780 - RNA, 20 nt, synthetic construct
  source 1..20: mol_type = other RNA
ccaagaaaggccaggcgcgg

SEQ ID NO: 15781 - RNA, 20 nt, synthetic construct
  source 1..20: mol_type = other RNA
tatccaagaaaggccaggcg

SEQ ID NO: 15782 - RNA, 20 nt, synthetic construct
  source 1..20: mol_type = other RNA
ataaatatccaagaaaggcc

SEQ ID NO: 15783 - RNA, 20 nt, synthetic construct
  source 1..20: mol_type = other RNA
ggttaataaatatccaagaa

SEQ ID NO: 15784 - RNA, 20 nt, synthetic construct
  source 1..20: mol_type = other RNA
attattttttaaaagtctga

SEQ ID NO: 15785 - RNA, 20 nt, synthetic construct
  source 1..20: mol_type = other RNA
gacttttaaaaaataatccc

SEQ ID NO: 15786 - RNA, 20 nt, synthetic construct
  source 1..20: mol_type = other RNA
acttttaaaaaataatccca

SEQ ID NO: 15787 - RNA, 20 nt, synthetic construct
  source 1..20: mol_type = other RNA
ggcagaattgtatcttccct

SEQ ID NO: 15788 - RNA, 20 nt, synthetic construct
  source 1..20: mol_type = other RNA
gggcagaattgtatcttccc

SEQ ID NO: 15789 - RNA, 20 nt, synthetic construct
  source 1..20: mol_type = other RNA
ggtatagtaaaggtctctga

SEQ ID NO: 15790 - RNA, 20 nt, synthetic construct
  source 1..20: mol_type = other RNA
tggtatagtaaaggtctctg

SEQ ID NO: 15791 - RNA, 20 nt, synthetic construct
  source 1..20: mol_type = other RNA
gtttggcaatggtatagtaa

SEQ ID NO: 15792 - RNA, 20 nt, synthetic construct
  source 1..20: mol_type = other RNA
tgggaaactgggtttggcaa

SEQ ID NO: 15793 - RNA, 20 nt, synthetic construct
  source 1..20: mol_type = other RNA
agcaagtgggaaactgggtt

SEQ ID NO: 15794 - RNA, 20 nt, synthetic construct
  source 1..20: mol_type = other RNA
cagtttcccacttgctccta

SEQ ID NO: 15795 - RNA, 20 nt, synthetic construct
  source 1..20: mol_type = other RNA
gtaggagcaagtgggaaact

SEQ ID NO: 15796 - RNA, 20 nt, synthetic construct
  source 1..20: mol_type = other RNA
cgtaggagcaagtgggaaac

SEQ ID NO: 15797 - RNA, 20 nt, synthetic construct
  source 1..20: mol_type = other RNA
ggaactccgtaggagcaagt

SEQ ID NO: 15798 - RNA, 20 nt, synthetic construct
  source 1..20: mol_type = other RNA
gggaactccgtaggagcaag

SEQ ID NO: 15799 - RNA, 20 nt, synthetic construct
  source 1..20: mol_type = other RNA
gtgggagctgggaactccgt

SEQ ID NO: 15800 - RNA, 20 nt, synthetic construct
  source 1..20: mol_type = other RNA
tagggcttcgtgtgggagct

SEQ ID NO: 15801 - RNA, 20 nt, synthetic construct
  source 1..20: mol_type = other RNA
atagggcttcgtgtgggagc

SEQ ID NO: 15802 - RNA, 20 nt, synthetic construct
  source 1..20: mol_type = other RNA
acacgaagccctatgtgcac

SEQ ID NO: 15803 - RNA, 20 nt, synthetic construct
  source 1..20: mol_type = other RNA
gtgcacatagggcttcgtgt

SEQ ID NO: 15804 - RNA, 20 nt, synthetic construct
  source 1..20: mol_type = other RNA
agtgcacatagggcttcgtg

SEQ ID NO: 15805 - RNA, 20 nt, synthetic construct
  source 1..20: mol_type = other RNA
tcttctgaccagtgcacata

SEQ ID NO: 15806 - RNA, 20 nt, synthetic construct
  source 1..20: mol_type = other RNA
gtcttctgaccagtgcacat

SEQ ID NO: 15807 - RNA, 20 nt, synthetic construct
  source 1..20: mol_type = other RNA
ccctgtcgtgttgtccccag

SEQ ID NO: 15808 - RNA, 20 nt, synthetic construct
  source 1..20: mol_type = other RNA
cctgtcgtgttgtccccaga

SEQ ID NO: 15809 - RNA, 20 nt, synthetic construct
  source 1..20: mol_type = other RNA
cctctggggacaacacgaca

SEQ ID NO: 15810 - RNA, 20 nt, synthetic construct
  source 1..20: mol_type = other RNA
ccctctggggacaacacgac

SEQ ID NO: 15811 - RNA, 20 nt, synthetic construct
  source 1..20: mol_type = other RNA
gactggcgccatgccctctg

SEQ ID NO: 15812 - RNA, 20 nt, synthetic construct
  source 1..20: mol_type = other RNA
tgactggcgccatgccctct

SEQ ID NO: 15813 - RNA, 20 nt, synthetic construct
  source 1..20: mol_type = other RNA
gtgactggcgccatgccctc

SEQ ID NO: 15814 - RNA, 20 nt, synthetic construct
  source 1..20: mol_type = other RNA
ctacagtaaactcaagtgac

SEQ ID NO: 15815 - RNA, 20 nt, synthetic construct
  source 1..20: mol_type = other RNA
cgcagccaccagccctgatg

SEQ ID NO: 15816 - RNA, 20 nt, synthetic construct
  source 1..20: mol_type = other RNA
gcagccaccagccctgatga

SEQ ID NO: 15817 - RNA, 20 nt, synthetic construct
  source 1..20: mol_type = other RNA
tcatcagggctggtggctgc

SEQ ID NO: 15818 - RNA, 20 nt, synthetic construct
  source 1..20: mol_type = other RNA
ctcatcagggctggtggctg

SEQ ID NO: 15819 - RNA, 20 nt, synthetic construct
  source 1..20: mol_type = other RNA
cagtccctcatcagggctgg

SEQ ID NO: 15820 - RNA, 20 nt, synthetic construct
  source 1..20: mol_type = other RNA
cagcagtccctcatcagggc

SEQ ID NO: 15821 - RNA, 20 nt, synthetic construct
  source 1..20: mol_type = other RNA
gactcagcagtccctcatca

SEQ ID NO: 15822 - RNA, 20 nt, synthetic construct
  source 1..20: mol_type = other RNA
tgactcagcagtccctcatc

SEQ ID NO: 15823 - RNA, 20 nt, synthetic construct
  source 1..20: mol_type = other RNA
tgagtcagagaagttagaac

SEQ ID NO: 15824 - RNA, 20 nt, synthetic construct
  source 1..20: mol_type = other RNA
gtcagagaagttagaacagg

SEQ ID NO: 15825 - RNA, 20 nt, synthetic construct
  source 1..20: mol_type = other RNA
tcagagaagttagaacagga

SEQ ID NO: 15826 - RNA, 20 nt, synthetic construct
  source 1..20: mol_type = other RNA
gattacagtgattattcaaa

SEQ ID NO: 15827 - RNA, 20 nt, synthetic construct
  source 1..20: mol_type = other RNA
ggattacagtgattattcaa

SEQ ID NO: 15828 - RNA, 20 nt, synthetic construct
  source 1..20: mol_type = other RNA
taatccctctcaacttagag

SEQ ID NO: 15829 - RNA, 20 nt, synthetic construct
  source 1..20: mol_type = other RNA
cagtccgctctaagttgaga

SEQ ID NO: 15830 - RNA, 20 nt, synthetic construct
  source 1..20: mol_type = other RNA
tcagtccgctctaagttgag

SEQ ID NO: 15831 - RNA, 20 nt, synthetic construct
  source 1..20: mol_type = other RNA
gcggactgagaaattgccca

SEQ ID NO: 15832 - RNA, 20 nt, synthetic construct
  source 1..20: mol_type = other RNA
cggactgagaaattgcccat

SEQ ID NO: 15833 - RNA, 20 nt, synthetic construct
  source 1..20: mol_type = other RNA
catgggctccataaaaaatg

SEQ ID NO: 15834 - RNA, 20 nt, synthetic construct
  source 1..20: mol_type = other RNA
acattttttatggagcccat

SEQ ID NO: 15835 - RNA, 20 nt, synthetic construct
  source 1..20: mol_type = other RNA
cacattttttatggagccca

SEQ ID NO: 15836 - RNA, 20 nt, synthetic construct
  source 1..20: mol_type = other RNA
ttcactgaccacatttttta

SEQ ID NO: 15837 - RNA, 20 nt, synthetic construct
  source 1..20: mol_type = other RNA
gtggtcagtgaacctatcga

SEQ ID NO: 15838 - RNA, 20 nt, synthetic construct
  source 1..20: mol_type = other RNA
tagtcttcatgtccttcgat

SEQ ID NO: 15839 - RNA, 20 nt, synthetic construct
  source 1..20: mol_type = other RNA
acatgaagactaccacatga

SEQ ID NO: 15840 - RNA, 20 nt, synthetic construct
  source 1..20: mol_type = other RNA
cacatgatggtaagtagcgc

SEQ ID NO: 15841 - RNA, 20 nt, synthetic construct
  source 1..20: mol_type = other RNA
cagcgctacttaccatcatg

SEQ ID NO: 15842 - RNA, 20 nt, synthetic construct
  source 1..20: mol_type = other RNA
aagtgggagtctagtgagag

SEQ ID NO: 15843 - RNA, 20 nt, synthetic construct
  source 1..20: mol_type = other RNA
gaagtgggagtctagtgaga

SEQ ID NO: 15844 - RNA, 20 nt, synthetic construct
  source 1..20: mol_type = other RNA
cactagactcccacttcacc

SEQ ID NO: 15845 - RNA, 20 nt, synthetic construct
  source 1..20: mol_type = other RNA
agactcccacttcacctggc

SEQ ID NO: 15846 - RNA, 20 nt, synthetic construct
  source 1..20: mol_type = other RNA
gactcccacttcacctggca

SEQ ID NO: 15847 - RNA, 20 nt, synthetic construct
  source 1..20: mol_type = other RNA
tgttccctgccaggtgaagt

SEQ ID NO: 15848 - RNA, 20 nt, synthetic construct
  source 1..20: mol_type = other RNA
ctgttccctgccaggtgaag

SEQ ID NO: 15849 - RNA, 20 nt, synthetic construct
  source 1..20: mol_type = other RNA
agttaaaactgttccctgcc

SEQ ID NO: 15850 - RNA, 20 nt, synthetic construct
  source 1..20: mol_type = other RNA
ttttaactgagcttgtttaa

SEQ ID NO: 15851 - RNA, 20 nt, synthetic construct
  source 1..20: mol_type = other RNA
ggatgtgagttaattaaaaa

SEQ ID NO: 15852 - RNA, 20 nt, synthetic construct
  source 1..20: mol_type = other RNA
gggatgtgagttaattaaaa

SEQ ID NO: 15853 - RNA, 20 nt, synthetic construct
  source 1..20: mol_type = other RNA
gacaaacatgggtgagggtt

SEQ ID NO: 15854 - RNA, 20 nt, synthetic construct
  source 1..20: mol_type = other RNA
ggacaaacatgggtgagggt

SEQ ID NO: 15855 - RNA, 20 nt, synthetic construct
  source 1..20: mol_type = other RNA
ggcaggacaaacatgggtga

SEQ ID NO: 15856 - RNA, 20 nt, synthetic construct
  source 1..20: mol_type = other RNA
aggcaggacaaacatgggtg

SEQ ID NO: 15857 - RNA, 20 nt, synthetic construct
  source 1..20: mol_type = other RNA
ccatgtttgtcctgcctgct

SEQ ID NO: 15858 - RNA, 20 nt, synthetic construct
  source 1..20: mol_type = other RNA
caagcaggcaggacaaacat

SEQ ID NO: 15859 - RNA, 20 nt, synthetic construct
  source 1..20: mol_type = other RNA
ccaagcaggcaggacaaaca

SEQ ID NO: 15860 - RNA, 20 nt, synthetic construct
  source 1..20: mol_type = other RNA
ggtcgggagaccaagcaggc

SEQ ID NO: 15861 - RNA, 20 nt, synthetic construct
  source 1..20: mol_type = other RNA
cagaggtcgggagaccaagc

SEQ ID NO: 15862 - RNA, 20 nt, synthetic construct
  source 1..20: mol_type = other RNA
ccgacctctgaagtaccgct

SEQ ID NO: 15863 - RNA, 20 nt, synthetic construct
  source 1..20: mol_type = other RNA
caagcggtacttcagaggtc

SEQ ID NO: 15864 - RNA, 20 nt, synthetic construct
  source 1..20: mol_type = other RNA
ccaagcggtacttcagaggt

SEQ ID NO: 15865 - RNA, 20 nt, synthetic construct
  source 1..20: mol_type = other RNA
aaaaccaagcggtacttcag

SEQ ID NO: 15866 - RNA, 20 nt, synthetic construct
  source 1..20: mol_type = other RNA
agggaaaaaggaaaaccaag

SEQ ID NO: 15867 - RNA, 20 nt, synthetic construct
  source 1..20: mol_type = other RNA
ggttttcctttttcccttcc

SEQ ID NO: 15868 - RNA, 20 nt, synthetic construct
  source 1..20: mol_type = other RNA
gaaacgcctggaagggaaaa

SEQ ID NO: 15869 - RNA, 20 nt, synthetic construct
  source 1..20: mol_type = other RNA
tcccttccaggcgtttcagt

SEQ ID NO: 15870 - RNA, 20 nt, synthetic construct
  source 1..20: mol_type = other RNA
cccttccaggcgtttcagtt

SEQ ID NO: 15871 - RNA, 20 nt, synthetic construct
  source 1..20: mol_type = other RNA
cccaactgaaacgcctggaa

SEQ ID NO: 15872 - RNA, 20 nt, synthetic construct
  source 1..20: mol_type = other RNA
gcccaactgaaacgcctgga

SEQ ID NO: 15873 - RNA, 20 nt, synthetic construct
  source 1..20: mol_type = other RNA
ggcgtttcagttgggcccca

SEQ ID NO: 15874 - RNA, 20 nt, synthetic construct
  source 1..20: mol_type = other RNA
tggggcccaactgaaacgcc

SEQ ID NO: 15875 - RNA, 20 nt, synthetic construct
  source 1..20: mol_type = other RNA
ccacggaagcctcttactac

SEQ ID NO: 15876 - RNA, 20 nt, synthetic construct
  source 1..20: mol_type = other RNA
cacggaagcctcttactact

SEQ ID NO: 15877 - RNA, 20 nt, synthetic construct
  source 1..20: mol_type = other RNA
agtagtaagaggcttccgtg

SEQ ID NO: 15878 - RNA, 20 nt, synthetic construct
  source 1..20: mol_type = other RNA
cagtagtaagaggcttccgt

SEQ ID NO: 15879 - RNA, 20 nt, synthetic construct
  source 1..20: mol_type = other RNA
ccagtagtaagaggcttccg

SEQ ID NO: 15880 - RNA, 20 nt, synthetic construct
  source 1..20: mol_type = other RNA
cctcttactactgggtgtac

SEQ ID NO: 15881 - RNA, 20 nt, synthetic construct
  source 1..20: mol_type = other RNA
ctcttactactgggtgtact

SEQ ID NO: 15882 - RNA, 20 nt, synthetic construct
  source 1..20: mol_type = other RNA
ccagtacacccagtagtaag

SEQ ID NO: 15883 - RNA, 20 nt, synthetic construct
  source 1..20: mol_type = other RNA
ctgggttccaactcaatatg

SEQ ID NO: 15884 - RNA, 20 nt, synthetic construct
  source 1..20: mol_type = other RNA
attgcatccacatattgagt

SEQ ID NO: 15885 - RNA, 20 nt, synthetic construct
  source 1..20: mol_type = other RNA
tgcaatcaaagacactgtgc

SEQ ID NO: 15886 - RNA, 20 nt, synthetic construct
  source 1..20: mol_type = other RNA
gcaatcaaagacactgtgct

SEQ ID NO: 15887 - RNA, 20 nt, synthetic construct
  source 1..20: mol_type = other RNA
caatcaaagacactgtgctg

SEQ ID NO: 15888 - RNA, 20 nt, synthetic construct
  source 1..20: mol_type = other RNA
aagacactgtgctggggaaa

SEQ ID NO: 15889 - RNA, 20 nt, synthetic construct
  source 1..20: mol_type = other RNA
tttgaaagcactttcacctc

SEQ ID NO: 15890 - RNA, 20 nt, synthetic construct
  source 1..20: mol_type = other RNA
agcactttcacctctggccc

SEQ ID NO: 15891 - RNA, 20 nt, synthetic construct
  source 1..20: mol_type = other RNA
gggtcagtctcctgggccag

SEQ ID NO: 15892 - RNA, 20 nt, synthetic construct
  source 1..20: mol_type = other RNA
aggagactgacccaaagtga

SEQ ID NO: 15893 - RNA, 20 nt, synthetic construct
  source 1..20: mol_type = other RNA
tcactttgggtcagtctcct

SEQ ID NO: 15894 - RNA, 20 nt, synthetic construct
  source 1..20: mol_type = other RNA
ttcactttgggtcagtctcc

SEQ ID NO: 15895 - RNA, 20 nt, synthetic construct
  source 1..20: mol_type = other RNA
cccaaagtgaaggacattgc

SEQ ID NO: 15896 - RNA, 20 nt, synthetic construct
  source 1..20: mol_type = other RNA
ccaaagtgaaggacattgcc

SEQ ID NO: 15897 - RNA, 20 nt, synthetic construct
  source 1..20: mol_type = other RNA
ccggcaatgtccttcacttt

SEQ ID NO: 15898 - RNA, 20 nt, synthetic construct
  source 1..20: mol_type = other RNA
gtgaaggacattgccgggag

SEQ ID NO: 15899 - RNA, 20 nt, synthetic construct
  source 1..20: mol_type = other RNA
ggagaggcctgcagcatccc

SEQ ID NO: 15900 - RNA, 20 nt, synthetic construct
  source 1..20: mol_type = other RNA
gggatgctgcaggcctctcc

SEQ ID NO: 15901 - RNA, 20 nt, synthetic construct
  source 1..20: mol_type = other RNA
ctgaaatccagggatgctgc

SEQ ID NO: 15902 - RNA, 20 nt, synthetic construct
  source 1..20: mol_type = other RNA
atccctggatttcagagttc

SEQ ID NO: 15903 - RNA, 20 nt, synthetic construct
  source 1..20: mol_type = other RNA
ttccagaactctgaaatcca

SEQ ID NO: 15904 - RNA, 20 nt, synthetic construct
  source 1..20: mol_type = other RNA
gttccagaactctgaaatcc

SEQ ID NO: 15905 - RNA, 20 nt, synthetic construct
  source 1..20: mol_type = other RNA
aaaaatctatattcaatctg

SEQ ID NO: 15906 - RNA, 20 nt, synthetic construct
  source 1..20: mol_type = other RNA
atattcaatctgaggtgatg

SEQ ID NO: 15907 - RNA, 20 nt, synthetic construct
  source 1..20: mol_type = other RNA
gatgtggtgactgaagccag

SEQ ID NO: 15908 - RNA, 20 nt, synthetic construct
  source 1..20: mol_type = other RNA
tggtgaaagtacatcacctc

SEQ ID NO: 15909 - RNA, 20 nt, synthetic construct
  source 1..20: mol_type = other RNA
ttaagttaaaattaagctaa

SEQ ID NO: 15910 - RNA, 20 nt, synthetic construct
  source 1..20: mol_type = other RNA
ctgactgcaagaaagggaac

SEQ ID NO: 15911 - RNA, 20 nt, synthetic construct
  source 1..20: mol_type = other RNA
atgaagctgactgcaagaaa

SEQ ID NO: 15912 - RNA, 20 nt, synthetic construct
  source 1..20: mol_type = other RNA
tatgaagctgactgcaagaa

SEQ ID NO: 15913 - RNA, 20 nt, synthetic construct
  source 1..20: mol_type = other RNA
catttttaaagtcaatacga

SEQ ID NO: 15914 - RNA, 20 nt, synthetic construct
  source 1..20: mol_type = other RNA
catcgtattgactttaaaaa

SEQ ID NO: 15915 - RNA, 20 nt, synthetic construct
  source 1..20: mol_type = other RNA
tgaattccgaacatgttgtg

SEQ ID NO: 15916 - RNA, 20 nt, synthetic construct
  source 1..20: mol_type = other RNA
agtattccacacaacatgtt

SEQ ID NO: 15917 - RNA, 20 nt, synthetic construct
  source 1..20: mol_type = other RNA
atctgccaattatgttgaca

SEQ ID NO: 15918 - RNA, 20 nt, synthetic construct
  source 1..20: mol_type = other RNA
tctgccaattatgttgacaa

SEQ ID NO: 15919 - RNA, 20 nt, synthetic construct
  source 1..20: mol_type = other RNA
cattcccttgtcaacataat

SEQ ID NO: 15920 - RNA, 20 nt, synthetic construct
  source 1..20: mol_type = other RNA
gaaatattttcatacatctt

SEQ ID NO: 15921 - RNA, 20 nt, synthetic construct
  source 1..20: mol_type = other RNA
catctttggttgcaaacatt

SEQ ID NO: 15922 - RNA, 20 nt, synthetic construct
  source 1..20: mol_type = other RNA
tggactgcattgcaatgagt

SEQ ID NO: 15923 - RNA, 20 nt, synthetic construct
  source 1..20: mol_type = other RNA
ggactgcattgcaatgagtt

SEQ ID NO: 15924 - RNA, 20 nt, synthetic construct
  source 1..20: mol_type = other RNA
gactgcattgcaatgagttg

SEQ ID NO: 15925 - RNA, 20 nt, synthetic construct
  source 1..20: mol_type = other RNA
catacaattttatacaaaaa

SEQ ID NO: 15926 - RNA, 20 nt, synthetic construct
  source 1..20: mol_type = other RNA
gtataaaattgtatgcaaaa

SEQ ID NO: 15927 - RNA, 20 nt, synthetic construct
  source 1..20: mol_type = other RNA
tataaaattgtatgcaaaat

SEQ ID NO: 15928 - RNA, 20 nt, synthetic construct
  source 1..20: mol_type = other RNA
ataaaattgtatgcaaaatg

SEQ ID NO: 15929 - RNA, 20 nt, synthetic construct
  source 1..20: mol_type = other RNA
taaaattgtatgcaaaatgg

SEQ ID NO: 15930 - RNA, 20 nt, synthetic construct
  source 1..20: mol_type = other RNA
aattgtatgcaaaatggggg

SEQ ID NO: 15931 - RNA, 20 nt, synthetic construct
  source 1..20: mol_type = other RNA
attgtatgcaaaatgggggt

SEQ ID NO: 15932 - RNA, 20 nt, synthetic construct
  source 1..20: mol_type = other RNA
aatcaatggacagaaatatg

SEQ ID NO: 15933 - RNA, 20 nt, synthetic construct
  source 1..20: mol_type = other RNA
aagaattaaatctgaatcaa

SEQ ID NO: 15934 - RNA, 20 nt, synthetic construct
  source 1..20: mol_type = other RNA
ggaagcgagagaatgaaaaa

SEQ ID NO: 15935 - RNA, 20 nt, synthetic construct
  source 1..20: mol_type = other RNA
aggaagcgagagaatgaaaa

SEQ ID NO: 15936 - RNA, 20 nt, synthetic construct
  source 1..20: mol_type = other RNA
taaaacaaaaactcaaattg

SEQ ID NO: 15937 - RNA, 20 nt, synthetic construct
  source 1..20: mol_type = other RNA
aaagatgtcagttcttcttt

SEQ ID NO: 15938 - RNA, 20 nt, synthetic construct
  source 1..20: mol_type = other RNA
aaagaagaactgacatcttt

SEQ ID NO: 15939 - RNA, 20 nt, synthetic construct
  source 1..20: mol_type = other RNA
aaaagaagaactgacatctt

SEQ ID NO: 15940 - RNA, 20 nt, synthetic construct
  source 1..20: mol_type = other RNA
ctcatcaacgcttcctttcc

SEQ ID NO: 15941 - RNA, 20 nt, synthetic construct
  source 1..20: mol_type = other RNA
tcatcaacgcttcctttcct

SEQ ID NO: 15942 - RNA, 20 nt, synthetic construct
  source 1..20: mol_type = other RNA
caggaaaggaagcgttgatg

SEQ ID NO: 15943 - RNA, 20 nt, synthetic construct
  source 1..20: mol_type = other RNA
ggcgggagggagcccaggaa

SEQ ID NO: 15944 - RNA, 20 nt, synthetic construct
  source 1..20: mol_type = other RNA
agcacggcgggagggagccc

SEQ ID NO: 15945 - RNA, 20 nt, synthetic construct
  source 1..20: mol_type = other RNA
gcagcagcagcacggcggga

SEQ ID NO: 15946 - RNA, 20 nt, synthetic construct
  source 1..20: mol_type = other RNA
ggcagcagcagcacggcggg

SEQ ID NO: 15947 - RNA, 20 nt, synthetic construct
  source 1..20: mol_type = other RNA
acaggcagcagcagcacggc

SEQ ID NO: 15948 - RNA, 20 nt, synthetic construct
  source 1..20: mol_type = other RNA
cacaggcagcagcagcacgg

SEQ ID NO: 15949 - RNA, 20 nt, synthetic construct
  source 1..20: mol_type = other RNA
gttcacaggcagcagcagca

SEQ ID NO: 15950 - RNA, 20 nt, synthetic construct
  source 1..20: mol_type = other RNA
tgctgctgcctgtgaacgca

SEQ ID NO: 15951 - RNA, 20 nt, synthetic construct
  source 1..20: mol_type = other RNA
tgctgcctgtgaacgcacgg

SEQ ID NO: 15952 - RNA, 20 nt, synthetic construct
  source 1..20: mol_type = other RNA
gctgcctgtgaacgcacggt

SEQ ID NO: 15953 - RNA, 20 nt, synthetic construct
  source 1..20: mol_type = other RNA
ctgtgaacgcacggtgggag

SEQ ID NO: 15954 - RNA, 20 nt, synthetic construct
  source 1..20: mol_type = other RNA
ctctcccaccgtgcgttcac

SEQ ID NO: 15955 - RNA, 20 nt, synthetic construct
  source 1..20: mol_type = other RNA
gaggaagagctgctcagtct

SEQ ID NO: 15956 - RNA, 20 nt, synthetic construct
  source 1..20: mol_type = other RNA
aggaagagctgctcagtctt

SEQ ID NO: 15957 - RNA, 20 nt, synthetic construct
  source 1..20: mol_type = other RNA
gagctgctcagtcttgggca

SEQ ID NO: 15958 - RNA, 20 nt, synthetic construct
  source 1..20: mol_type = other RNA
aggagctctcacacttgctg

SEQ ID NO: 15959 - RNA, 20 nt, synthetic construct
  source 1..20: mol_type = other RNA
acatttaaacaggagtcact

SEQ ID NO: 15960 - RNA, 20 nt, synthetic construct
  source 1..20: mol_type = other RNA
gacatttaaacaggagtcac

SEQ ID NO: 15961 - RNA, 20 nt, synthetic construct
  source 1..20: mol_type = other RNA
tgtttaaatgtcttgccctt

SEQ ID NO: 15962 - RNA, 20 nt, synthetic construct
  source 1..20: mol_type = other RNA
gtttaaatgtcttgcccttt

SEQ ID NO: 15963 - RNA, 20 nt, synthetic construct
  source 1..20: mol_type = other RNA
aaagggcaagacatttaaac

SEQ ID NO: 15964 - RNA, 20 nt, synthetic construct
  source 1..20: mol_type = other RNA
cctttgggcccccatctcca

SEQ ID NO: 15965 - RNA, 20 nt, synthetic construct
  source 1..20: mol_type = other RNA
cttggagatgggggcccaaa

SEQ ID NO: 15966 - RNA, 20 nt, synthetic construct
  source 1..20: mol_type = other RNA
ccttggagatgggggcccaa

SEQ ID NO: 15967 - RNA, 20 nt, synthetic construct
  source 1..20: mol_type = other RNA
atggaactccttggagatgg

SEQ ID NO: 15968 - RNA, 20 nt, synthetic construct
  source 1..20: mol_type = other RNA
tctccaaggagttccattgc

SEQ ID NO: 15969 - RNA, 20 nt, synthetic construct
  source 1..20: mol_type = other RNA
caatggaactccttggagat

SEQ ID NO: 15970 - RNA, 20 nt, synthetic construct
  source 1..20: mol_type = other RNA
gcaatggaactccttggaga

SEQ ID NO: 15971 - RNA, 20 nt, synthetic construct
  source 1..20: mol_type = other RNA
caaggagttccattgctggt

SEQ ID NO: 15972 - RNA, 20 nt, synthetic construct
  source 1..20: mol_type = other RNA
caaccagcaatggaactcct

SEQ ID NO: 15973 - RNA, 20 nt, synthetic construct
  source 1..20: mol_type = other RNA
gacaatcatccaaccagcaa

SEQ ID NO: 15974 - RNA, 20 nt, synthetic construct
  source 1..20: mol_type = other RNA
tctgcacccctcactgagct

SEQ ID NO: 15975 - RNA, 20 nt, synthetic construct
  source 1..20: mol_type = other RNA
cctcactgagcttggcctag

SEQ ID NO: 15976 - RNA, 20 nt, synthetic construct
  source 1..20: mol_type = other RNA
tctaggccaagctcagtgag

SEQ ID NO: 15977 - RNA, 20 nt, synthetic construct
  source 1..20: mol_type = other RNA
ctctaggccaagctcagtga

SEQ ID NO: 15978 - RNA, 20 nt, synthetic construct
  source 1..20: mol_type = other RNA
cctctaggccaagctcagtg

SEQ ID NO: 15979 - RNA, 20 nt, synthetic construct
  source 1..20: mol_type = other RNA
cttggcctagaggcccagcc

SEQ ID NO: 15980 - RNA, 20 nt, synthetic construct
  source 1..20: mol_type = other RNA
cctagaggcccagcctggca

SEQ ID NO: 15981 - RNA, 20 nt, synthetic construct
  source 1..20: mol_type = other RNA
ccatgccaggctgggcctct

SEQ ID NO: 15982 - RNA, 20 nt, synthetic construct
  source 1..20: mol_type = other RNA
cagcctggcatggttgtgcc

SEQ ID NO: 15983 - RNA, 20 nt, synthetic construct
  source 1..20: mol_type = other RNA
agcctggcatggttgtgcct

SEQ ID NO: 15984 - RNA, 20 nt, synthetic construct
  source 1..20: mol_type = other RNA
aggcacaaccatgccaggct

SEQ ID NO: 15985 - RNA, 20 nt, synthetic construct
  source 1..20: mol_type = other RNA
caggcacaaccatgccaggc

SEQ ID NO: 15986 - RNA, 20 nt, synthetic construct
  source 1..20: mol_type = other RNA
agcccaggcacaaccatgcc

SEQ ID NO: 15987 - RNA, 20 nt, synthetic construct
  source 1..20: mol_type = other RNA
gctgttgagcggcacagccc

SEQ ID NO: 15988 - RNA, 20 nt, synthetic construct
  source 1..20: mol_type = other RNA
tgggagctggggctgttgag

SEQ ID NO: 15989 - RNA, 20 nt, synthetic construct
  source 1..20: mol_type = other RNA
ctttgtctgcttgggagctg

SEQ ID NO: 15990 - RNA, 20 nt, synthetic construct
  source 1..20: mol_type = other RNA
tctttgtctgcttgggagct

SEQ ID NO: 15991 - RNA, 20 nt, synthetic construct
  source 1..20: mol_type = other RNA
gtctttgtctgcttgggagc

SEQ ID NO: 15992 - RNA, 20 nt, synthetic construct
  source 1..20: mol_type = other RNA
agcagacaaagacctcttcc

SEQ ID NO: 15993 - RNA, 20 nt, synthetic construct
  source 1..20: mol_type = other RNA
gaagaggtctttgtctgctt

SEQ ID NO: 15994 - RNA, 20 nt, synthetic construct
  source 1..20: mol_type = other RNA
ggaagaggtctttgtctgct

SEQ ID NO: 15995 - RNA, 20 nt, synthetic construct
  source 1..20: mol_type = other RNA
agacaaagacctcttccagg

SEQ ID NO: 15996 - RNA, 20 nt, synthetic construct
  source 1..20: mol_type = other RNA
gacctcttccaggaggagcc

SEQ ID NO: 15997 - RNA, 20 nt, synthetic construct
  source 1..20: mol_type = other RNA
tacctggctcctcctggaag

SEQ ID NO: 15998 - RNA, 20 nt, synthetic construct
  source 1..20: mol_type = other RNA
atcttctacctggctcctcc

SEQ ID NO: 15999 - RNA, 20 nt, synthetic construct
  source 1..20: mol_type = other RNA
ctgtataactatcttctacc

SEQ ID NO: 16000 - RNA, 20 nt, synthetic construct
  source 1..20: mol_type = other RNA
tatctggatctgcagctata

SEQ ID NO: 16001 - RNA, 20 nt, synthetic construct
  source 1..20: mol_type = other RNA
tccagataaccttctttctt

SEQ ID NO: 16002 - RNA, 20 nt, synthetic construct
  source 1..20: mol_type = other RNA
tccaaagaaagaaggttatc

SEQ ID NO: 16003 - RNA, 20 nt, synthetic construct
  source 1..20: mol_type = other RNA
tgaaaacttccaaagaaaga

SEQ ID NO: 16004 - RNA, 20 nt, synthetic construct
  source 1..20: mol_type = other RNA
agaaattcttaagcagtcca

SEQ ID NO: 16005 - RNA, 20 nt, synthetic construct
  source 1..20: mol_type = other RNA
agcataattgaaatcatcct

SEQ ID NO: 16006 - RNA, 20 nt, synthetic construct
  source 1..20: mol_type = other RNA
tttcaattatgcttctccat

SEQ ID NO: 16007 - RNA, 20 nt, synthetic construct
  source 1..20: mol_type = other RNA
ttcaattatgcttctccatt

SEQ ID NO: 16008 - RNA, 20 nt, synthetic construct
  source 1..20: mol_type = other RNA
gcatgagcagaaggacccaa

SEQ ID NO: 16009 - RNA, 20 nt, synthetic construct
  source 1..20: mol_type = other RNA
gaactgaatgcatgagcaga

SEQ ID NO: 16010 - RNA, 20 nt, synthetic construct
  source 1..20: mol_type = other RNA
gttcaagtgtcctttatccc

SEQ ID NO: 16011 - RNA, 20 nt, synthetic construct
  source 1..20: mol_type = other RNA
catctctgaacctgggataa

SEQ ID NO: 16012 - RNA, 20 nt, synthetic construct
  source 1..20: mol_type = other RNA
aaggcagcatctctgaacct

SEQ ID NO: 16013 - RNA, 20 nt, synthetic construct
  source 1..20: mol_type = other RNA
aaaggcagcatctctgaacc

SEQ ID NO: 16014 - RNA, 20 nt, synthetic construct
  source 1..20: mol_type = other RNA
gtcagatgtcttcttcagaa

SEQ ID NO: 16015 - RNA, 20 nt, synthetic construct
  source 1..20: mol_type = other RNA
agaagacatctgaccctagc

SEQ ID NO: 16016 - RNA, 20 nt, synthetic construct
  source 1..20: mol_type = other RNA
gacatctgaccctagcaggt

SEQ ID NO: 16017 - RNA, 20 nt, synthetic construct
  source 1..20: mol_type = other RNA
taacactggccaacctgcta

SEQ ID NO: 16018 - RNA, 20 nt, synthetic construct
  source 1..20: mol_type = other RNA
ataacactggccaacctgct

SEQ ID NO: 16019 - RNA, 20 nt, synthetic construct
  source 1..20: mol_type = other RNA
gtgttattgaacaacaaaaa

SEQ ID NO: 16020 - RNA, 20 nt, synthetic construct
  source 1..20: mol_type = other RNA
tgttattgaacaacaaaaat

SEQ ID NO: 16021 - RNA, 20 nt, synthetic construct
  source 1..20: mol_type = other RNA
tttttgttgttcaataacac

SEQ ID NO: 16022 - RNA, 20 nt, synthetic construct
  source 1..20: mol_type = other RNA
atgattagctcaccttcttc

SEQ ID NO: 16023 - RNA, 20 nt, synthetic construct
  source 1..20: mol_type = other RNA
gaagggctaaaaccagaaga

SEQ ID NO: 16024 - RNA, 20 nt, synthetic construct
  source 1..20: mol_type = other RNA
cacgtgtacagagaacagaa

SEQ ID NO: 16025 - RNA, 20 nt, synthetic construct
  source 1..20: mol_type = other RNA
tcacgtgtacagagaacaga

SEQ ID NO: 16026 - RNA, 20 nt, synthetic construct
  source 1..20: mol_type = other RNA
gaacttctgtcatctccttc

SEQ ID NO: 16027 - RNA, 20 nt, synthetic construct
  source 1..20: mol_type = other RNA
tctgtcatctccttctggct

SEQ ID NO: 16028 - RNA, 20 nt, synthetic construct
  source 1..20: mol_type = other RNA
ctggcttggttgcctctgaa

SEQ ID NO: 16029 - RNA, 20 nt, synthetic construct
  source 1..20: mol_type = other RNA
tcagaggcaaccaagccaga

SEQ ID NO: 16030 - RNA, 20 nt, synthetic construct
  source 1..20: mol_type = other RNA
gcttggttgcctctgaaagg

SEQ ID NO: 16031 - RNA, 20 nt, synthetic construct
  source 1..20: mol_type = other RNA
cttggttgcctctgaaagga

SEQ ID NO: 16032 - RNA, 20 nt, synthetic construct
  source 1..20: mol_type = other RNA
tgaaaggagggaaagtctct

SEQ ID NO: 16033 - RNA, 20 nt, synthetic construct
  source 1..20: mol_type = other RNA
gagactttccctcctttcag

SEQ ID NO: 16034 - RNA, 20 nt, synthetic construct
  source 1..20: mol_type = other RNA
ctttgcagttctcctctcac

SEQ ID NO: 16035 - RNA, 20 nt, synthetic construct
  source 1..20: mol_type = other RNA
tgagaggagaactgcaaaga

SEQ ID NO: 16036 - RNA, 20 nt, synthetic construct
  source 1..20: mol_type = other RNA
gttctcctctcactggttgc

SEQ ID NO: 16037 - RNA, 20 nt, synthetic construct
  source 1..20: mol_type = other RNA
gaaagcctgcaaccagtgag

SEQ ID NO: 16038 - RNA, 20 nt, synthetic construct
  source 1..20: mol_type = other RNA
ggttgcaggctttcatagta

SEQ ID NO: 16039 - RNA, 20 nt, synthetic construct
  source 1..20: mol_type = other RNA
caggctttcatagtaaggtt

SEQ ID NO: 16040 - RNA, 20 nt, synthetic construct
  source 1..20: mol_type = other RNA
atgttccaaacatcacattt

SEQ ID NO: 16041 - RNA, 20 nt, synthetic construct
  source 1..20: mol_type = other RNA
aacatcacattttggattct

SEQ ID NO: 16042 - RNA, 20 nt, synthetic construct
  source 1..20: mol_type = other RNA
agaatccaaaatgtgatgtt

SEQ ID NO: 16043 - RNA, 20 nt, synthetic construct
  source 1..20: mol_type = other RNA
aatacgtttcacagaatgag

SEQ ID NO: 16044 - RNA, 20 nt, synthetic construct
  source 1..20: mol_type = other RNA
taatacgtttcacagaatga

SEQ ID NO: 16045 - RNA, 20 nt, synthetic construct
  source 1..20: mol_type = other RNA
ctaatacgtttcacagaatg

SEQ ID NO: 16046 - RNA, 20 nt, synthetic construct
  source 1..20: mol_type = other RNA
tcacaaggaatagtcatctt

SEQ ID NO: 16047 - RNA, 20 nt, synthetic construct
  source 1..20: mol_type = other RNA
ctcacaaggaatagtcatct

SEQ ID NO: 16048 - RNA, 20 nt, synthetic construct
  source 1..20: mol_type = other RNA
tcatcattaactggctcaca

SEQ ID NO: 16049 - RNA, 20 nt, synthetic construct
  source 1..20: mol_type = other RNA
cgtagaatatcatcattaac

SEQ ID NO: 16050 - RNA, 20 nt, synthetic construct
  source 1..20: mol_type = other RNA
tcccttctaagctgtagttc

SEQ ID NO: 16051 - RNA, 20 nt, synthetic construct
  source 1..20: mol_type = other RNA
aactacagcttagaagggaa

SEQ ID NO: 16052 - RNA, 20 nt, synthetic construct
  source 1..20: mol_type = other RNA
gaactacagcttagaaggga

SEQ ID NO: 16053 - RNA, 20 nt, synthetic construct
  source 1..20: mol_type = other RNA
tcctgaactacagcttagaa

SEQ ID NO: 16054 - RNA, 20 nt, synthetic construct
  source 1..20: mol_type = other RNA
ttcctgaactacagcttaga

SEQ ID NO: 16055 - RNA, 20 nt, synthetic construct
  source 1..20: mol_type = other RNA
aagagtctgtctatgtgggc

SEQ ID NO: 16056 - RNA, 20 nt, synthetic construct
  source 1..20: mol_type = other RNA
aagcaagagtctgtctatgt

SEQ ID NO: 16057 - RNA, 20 nt, synthetic construct
  source 1..20: mol_type = other RNA
aaagcaagagtctgtctatg

SEQ ID NO: 16058 - RNA, 20 nt, synthetic construct
  source 1..20: mol_type = other RNA
agacagactcttgctttcca

SEQ ID NO: 16059 - RNA, 20 nt, synthetic construct
  source 1..20: mol_type = other RNA
acttggcattgactacacca

SEQ ID NO: 16060 - RNA, 20 nt, synthetic construct
  source 1..20: mol_type = other RNA
caatgccaagtgatgcatct

SEQ ID NO: 16061 - RNA, 20 nt, synthetic construct
  source 1..20: mol_type = other RNA
gccaagtgatgcatctaggc

SEQ ID NO: 16062 - RNA, 20 nt, synthetic construct
  source 1..20: mol_type = other RNA
tcctgcctagatgcatcact

SEQ ID NO: 16063 - RNA, 20 nt, synthetic construct
  source 1..20: mol_type = other RNA
aaatctactctttgcttttt

SEQ ID NO: 16064 - RNA, 20 nt, synthetic construct
  source 1..20: mol_type = other RNA
aatctactctttgctttttt

SEQ ID NO: 16065 - RNA, 20 nt, synthetic construct
  source 1..20: mol_type = other RNA
atctactctttgcttttttg

SEQ ID NO: 16066 - RNA, 20 nt, synthetic construct
  source 1..20: mol_type = other RNA
tctactctttgcttttttgg

SEQ ID NO: 16067 - RNA, 20 nt, synthetic construct
  source 1..20: mol_type = other RNA
tgaaaaaacaggctgtttct

SEQ ID NO: 16068 - RNA, 20 nt, synthetic construct
  source 1..20: mol_type = other RNA
gttttttcatcccttgagaa

SEQ ID NO: 16069 - RNA, 20 nt, synthetic construct
  source 1..20: mol_type = other RNA
ttctcaagggatgaaaaaac

SEQ ID NO: 16070 - RNA, 20 nt, synthetic construct
  source 1..20: mol_type = other RNA
aatgactgctcctttctcaa

SEQ ID NO: 16071 - RNA, 20 nt, synthetic construct
  source 1..20: mol_type = other RNA
caatgactgctcctttctca

SEQ ID NO: 16072 - RNA, 20 nt, synthetic construct
  source 1..20: mol_type = other RNA
tgcagcttttctgtccttgt

SEQ ID NO: 16073 - RNA, 20 nt, synthetic construct
  source 1..20: mol_type = other RNA
ccttgtcggcctgcagttcc

SEQ ID NO: 16074 - RNA, 20 nt, synthetic construct
  source 1..20: mol_type = other RNA
cttgtcggcctgcagttcct

SEQ ID NO: 16075 - RNA, 20 nt, synthetic construct
  source 1..20: mol_type = other RNA
ttgtcggcctgcagttcctg

SEQ ID NO: 16076 - RNA, 20 nt, synthetic construct
  source 1..20: mol_type = other RNA
ccaggaactgcaggccgaca

SEQ ID NO: 16077 - RNA, 20 nt, synthetic construct
  source 1..20: mol_type = other RNA
ctcttttccccaggaactgc

SEQ ID NO: 16078 - RNA, 20 nt, synthetic construct
  source 1..20: mol_type = other RNA
tcagatgtactcttttcccc

SEQ ID NO: 16079 - RNA, 20 nt, synthetic construct
  source 1..20: mol_type = other RNA
ttgtccaagcctctgtctgc

SEQ ID NO: 16080 - RNA, 20 nt, synthetic construct
  source 1..20: mol_type = other RNA
agcctctgtctgcaggtgac

SEQ ID NO: 16081 - RNA, 20 nt, synthetic construct
  source 1..20: mol_type = other RNA
gtcacctgcagacagaggct

SEQ ID NO: 16082 - RNA, 20 nt, synthetic construct
  source 1..20: mol_type = other RNA
tgtctgcaggtgacaggttt

SEQ ID NO: 16083 - RNA, 20 nt, synthetic construct
  source 1..20: mol_type = other RNA
gtctgcaggtgacaggtttt

SEQ ID NO: 16084 - RNA, 20 nt, synthetic construct
  source 1..20: mol_type = other RNA
tctgcaggtgacaggttttg

SEQ ID NO: 16085 - RNA, 20 nt, synthetic construct
  source 1..20: mol_type = other RNA
ctgcaggtgacaggttttgg

SEQ ID NO: 16086 - RNA, 20 nt, synthetic construct
  source 1..20: mol_type = other RNA
cattaagtagaacatcatct

SEQ ID NO: 16087 - RNA, 20 nt, synthetic construct
  source 1..20: mol_type = other RNA
attaagtagaacatcatctc

SEQ ID NO: 16088 - RNA, 20 nt, synthetic construct
  source 1..20: mol_type = other RNA
ggggcattggcaaacaaaag

SEQ ID NO: 16089 - RNA, 20 nt, synthetic construct
  source 1..20: mol_type = other RNA
tggggcattggcaaacaaaa

SEQ ID NO: 16090 - RNA, 20 nt, synthetic construct
  source 1..20: mol_type = other RNA
ctggggcattggcaaacaaa

SEQ ID NO: 16091 - RNA, 20 nt, synthetic construct
  source 1..20: mol_type = other RNA
agtctctaggactggggcat

SEQ ID NO: 16092 - RNA, 20 nt, synthetic construct
  source 1..20: mol_type = other RNA
aggacaagtctctaggactg

SEQ ID NO: 16093 - RNA, 20 nt, synthetic construct
  source 1..20: mol_type = other RNA
caggacaagtctctaggact

SEQ ID NO: 16094 - RNA, 20 nt, synthetic construct
  source 1..20: mol_type = other RNA
tcaggacaagtctctaggac

SEQ ID NO: 16095 - RNA, 20 nt, synthetic construct
  source 1..20: mol_type = other RNA
cactgtcaggacaagtctct

SEQ ID NO: 16096 - RNA, 20 nt, synthetic construct
  source 1..20: mol_type = other RNA
agtaggtgtgcggcactgtc

SEQ ID NO: 16097 - RNA, 20 nt, synthetic construct
  source 1..20: mol_type = other RNA
agagatcaaaagtaggtgtg

SEQ ID NO: 16098 - RNA, 20 nt, synthetic construct
  source 1..20: mol_type = other RNA
tacttttgatctctcagagc

SEQ ID NO: 16099 - RNA, 20 nt, synthetic construct
  source 1..20: mol_type = other RNA
ttttgatctctcagagcagg

SEQ ID NO: 16100 - RNA, 20 nt, synthetic construct
  source 1..20: mol_type = other RNA
gctccatccccagactagcc

SEQ ID NO: 16101 - RNA, 20 nt, synthetic construct
  source 1..20: mol_type = other RNA
cagccaggctagtctgggga

SEQ ID NO: 16102 - RNA, 20 nt, synthetic construct
  source 1..20: mol_type = other RNA
agagcagccaggctagtctg

SEQ ID NO: 16103 - RNA, 20 nt, synthetic construct
  source 1..20: mol_type = other RNA
gagagcagccaggctagtct

SEQ ID NO: 16104 - RNA, 20 nt, synthetic construct
  source 1..20: mol_type = other RNA
ggagagcagccaggctagtc

SEQ ID NO: 16105 - RNA, 20 nt, synthetic construct
  source 1..20: mol_type = other RNA
aggggcctcggagagcagcc

SEQ ID NO: 16106 - RNA, 20 nt, synthetic construct
  source 1..20: mol_type = other RNA
gggagcaggtggaggggcct

SEQ ID NO: 16107 - RNA, 20 nt, synthetic construct
  source 1..20: mol_type = other RNA
aataaggggagcaggtggag

SEQ ID NO: 16108 - RNA, 20 nt, synthetic construct
  source 1..20: mol_type = other RNA
caataaggggagcaggtgga

SEQ ID NO: 16109 - RNA, 20 nt, synthetic construct
  source 1..20: mol_type = other RNA
gcaataaggggagcaggtgg

SEQ ID NO: 16110 - RNA, 20 nt, synthetic construct
  source 1..20: mol_type = other RNA
ggggcaataaggggagcagg

SEQ ID NO: 16111 - RNA, 20 nt, synthetic construct
  source 1..20: mol_type = other RNA
aatggggcaataaggggagc

SEQ ID NO: 16112 - RNA, 20 nt, synthetic construct
  source 1..20: mol_type = other RNA
cccttattgccccattcttg

SEQ ID NO: 16113 - RNA, 20 nt, synthetic construct
  source 1..20: mol_type = other RNA
cacaagaatggggcaataag

SEQ ID NO: 16114 - RNA, 20 nt, synthetic construct
  source 1..20: mol_type = other RNA
ccacaagaatggggcaataa

SEQ ID NO: 16115 - RNA, 20 nt, synthetic construct
  source 1..20: mol_type = other RNA
gccacaagaatggggcaata

SEQ ID NO: 16116 - RNA, 20 nt, synthetic construct
  source 1..20: mol_type = other RNA
gccccattcttgtggcttgc

SEQ ID NO: 16117 - RNA, 20 nt, synthetic construct
  source 1..20: mol_type = other RNA
ccccattcttgtggcttgcc

SEQ ID NO: 16118 - RNA, 20 nt, synthetic construct
  source 1..20: mol_type = other RNA
cccggcaagccacaagaatg

SEQ ID NO: 16119 - RNA, 20 nt, synthetic construct
  source 1..20: mol_type = other RNA
gcccggcaagccacaagaat

SEQ ID NO: 16120 - RNA, 20 nt, synthetic construct
  source 1..20: mol_type = other RNA
ggcccggcaagccacaagaa

SEQ ID NO: 16121 - RNA, 20 nt, synthetic construct
  source 1..20: mol_type = other RNA
ttgtggcttgccgggccact

SEQ ID NO: 16122 - RNA, 20 nt, synthetic construct
  source 1..20: mol_type = other RNA
agaagggaggccaagtggcc

SEQ ID NO: 16123 - RNA, 20 nt, synthetic construct
  source 1..20: mol_type = other RNA
cacttggcctcccttcttgc

SEQ ID NO: 16124 - RNA, 20 nt, synthetic construct
  source 1..20: mol_type = other RNA
cggcaagaagggaggccaag

SEQ ID NO: 16125 - RNA, 20 nt, synthetic construct
  source 1..20: mol_type = other RNA
gctgtcaccggcaagaaggg

SEQ ID NO: 16126 - RNA, 20 nt, synthetic construct
  source 1..20: mol_type = other RNA
aacgctgtcaccggcaagaa

SEQ ID NO: 16127 - RNA, 20 nt, synthetic construct
  source 1..20: mol_type = other RNA
gaacgctgtcaccggcaaga

SEQ ID NO: 16128 - RNA, 20 nt, synthetic construct
  source 1..20: mol_type = other RNA
agatgatggaacgctgtcac

SEQ ID NO: 16129 - RNA, 20 nt, synthetic construct
  source 1..20: mol_type = other RNA
catcatctccccgctcccca

SEQ ID NO: 16130 - RNA, 20 nt, synthetic construct
  source 1..20: mol_type = other RNA
atcatctccccgctccccaa

SEQ ID NO: 16131 - RNA, 20 nt, synthetic construct
  source 1..20: mol_type = other RNA
cttggggagcggggagatga

SEQ ID NO: 16132 - RNA, 20 nt, synthetic construct
  source 1..20: mol_type = other RNA
cagttggcccttggggagcg

SEQ ID NO: 16133 - RNA, 20 nt, synthetic construct
  source 1..20: mol_type = other RNA
gcagttggcccttggggagc

SEQ ID NO: 16134 - RNA, 20 nt, synthetic construct
  source 1..20: mol_type = other RNA
agcagttggcccttggggag

SEQ ID NO: 16135 - RNA, 20 nt, synthetic construct
  source 1..20: mol_type = other RNA
tgagaagcagttggcccttg

SEQ ID NO: 16136 - RNA, 20 nt, synthetic construct
  source 1..20: mol_type = other RNA
gggccaactgcttctcactc

SEQ ID NO: 16137 - RNA, 20 nt, synthetic construct
  source 1..20: mol_type = other RNA
agtgagaagcagttggccct

SEQ ID NO: 16138 - RNA, 20 nt, synthetic construct
  source 1..20: mol_type = other RNA
caactgcttctcactcaggc

SEQ ID NO: 16139 - RNA, 20 nt, synthetic construct
  source 1..20: mol_type = other RNA
cagcctgagtgagaagcagt

SEQ ID NO: 16140 - RNA, 20 nt, synthetic construct
  source 1..20: mol_type = other RNA
actcaggctggtgtcatttc

SEQ ID NO: 16141 - RNA, 20 nt, synthetic construct
  source 1..20: mol_type = other RNA
caggctggtgtcatttcagg

SEQ ID NO: 16142 - RNA, 20 nt, synthetic construct
  source 1..20: mol_type = other RNA
aaaaaggctcacgcaggctt

SEQ ID NO: 16143 - RNA, 20 nt, synthetic construct
  source 1..20: mol_type = other RNA
gaaaataaaaaggctcacgc

SEQ ID NO: 16144 - RNA, 20 nt, synthetic construct
  source 1..20: mol_type = other RNA
cctttttattttcagtaaaa

SEQ ID NO: 16145 - RNA, 20 nt, synthetic construct
  source 1..20: mol_type = other RNA
ccattttactgaaaataaaa

SEQ ID NO: 16146 - RNA, 20 nt, synthetic construct
  source 1..20: mol_type = other RNA
atatatagtatctcgaagta

SEQ ID NO: 16147 - RNA, 20 nt, synthetic construct
  source 1..20: mol_type = other RNA
gtaaatgacaccttttcgta

SEQ ID NO: 16148 - RNA, 20 nt, synthetic construct
  source 1..20: mol_type = other RNA
tcaaacagctccgtacgaaa

SEQ ID NO: 16149 - RNA, 20 nt, synthetic construct
  source 1..20: mol_type = other RNA
ttcaacaatcttgagctctg

SEQ ID NO: 16150 - RNA, 20 nt, synthetic construct
  source 1..20: mol_type = other RNA
ggctcctcaccctgtctgca

SEQ ID NO: 16151 - RNA, 20 nt, synthetic construct
  source 1..20: mol_type = other RNA
tcttccatgcagacagggtg

SEQ ID NO: 16152 - RNA, 20 nt, synthetic construct
  source 1..20: mol_type = other RNA
gtctgcatggaagaccttgc

SEQ ID NO: 16153 - RNA, 20 nt, synthetic construct
  source 1..20: mol_type = other RNA
caaggtcttccatgcagaca

SEQ ID NO: 16154 - RNA, 20 nt, synthetic construct
  source 1..20: mol_type = other RNA
gcaaggtcttccatgcagac

SEQ ID NO: 16155 - RNA, 20 nt, synthetic construct
  source 1..20: mol_type = other RNA
aagaccttgctggacgctct

SEQ ID NO: 16156 - RNA, 20 nt, synthetic construct
  source 1..20: mol_type = other RNA
agaccttgctggacgctctc

SEQ ID NO: 16157 - RNA, 20 nt, synthetic construct
  source 1..20: mol_type = other RNA
tctcccgagagcgtccagca

SEQ ID NO: 16158 - RNA, 20 nt, synthetic construct
  source 1..20: mol_type = other RNA
gacatagcaccagaagccac

SEQ ID NO: 16159 - RNA, 20 nt, synthetic construct
  source 1..20: mol_type = other RNA
acatagcaccagaagccact

SEQ ID NO: 16160 - RNA, 20 nt, synthetic construct
  source 1..20: mol_type = other RNA
acacttctcccagtggcttc

SEQ ID NO: 16161 - RNA, 20 nt, synthetic construct
  source 1..20: mol_type = other RNA
atcgaaaacacttctcccag

SEQ ID NO: 16162 - RNA, 20 nt, synthetic construct
  source 1..20: mol_type = other RNA
aagtgttttcgatccgtgtc

SEQ ID NO: 16163 - RNA, 20 nt, synthetic construct
  source 1..20: mol_type = other RNA
agtgttttcgatccgtgtct

SEQ ID NO: 16164 - RNA, 20 nt, synthetic construct
  source 1..20: mol_type = other RNA
atactactgtggcccagaca

SEQ ID NO: 16165 - RNA, 20 nt, synthetic construct
  source 1..20: mol_type = other RNA
ctaaacagtgaatactactg

SEQ ID NO: 16166 - RNA, 20 nt, synthetic construct
  source 1..20: mol_type = other RNA
atgtatgaagagactgctta

SEQ ID NO: 16167 - RNA, 20 nt, synthetic construct
  source 1..20: mol_type = other RNA
ttcatacatttcttacagtc

SEQ ID NO: 16168 - RNA, 20 nt, synthetic construct
  source 1..20: mol_type = other RNA
attgaaatactctttctttt

SEQ ID NO: 16169 - RNA, 20 nt, synthetic construct
  source 1..20: mol_type = other RNA
tcttttaggtagcgtcacag

SEQ ID NO: 16170 - RNA, 20 nt, synthetic construct
  source 1..20: mol_type = other RNA
cagtggttttttttttcctc

SEQ ID NO: 16171 - RNA, 20 nt, synthetic construct
  source 1..20: mol_type = other RNA
attgtatagaaattatcctg

SEQ ID NO: 16172 - RNA, 20 nt, synthetic construct
  source 1..20: mol_type = other RNA
tacaatttccttactgtcag

SEQ ID NO: 16173 - RNA, 20 nt, synthetic construct
  source 1..20: mol_type = other RNA
acaatttccttactgtcaga

SEQ ID NO: 16174 - RNA, 20 nt, synthetic construct
  source 1..20: mol_type = other RNA
atctggtccctctgacagta

SEQ ID NO: 16175 - RNA, 20 nt, synthetic construct
  source 1..20: mol_type = other RNA
accagatctttccctcactg

SEQ ID NO: 16176 - RNA, 20 nt, synthetic construct
  source 1..20: mol_type = other RNA
gatctttccctcactgtggc

SEQ ID NO: 16177 - RNA, 20 nt, synthetic construct
  source 1..20: mol_type = other RNA
atctttccctcactgtggca

SEQ ID NO: 16178 - RNA, 20 nt, synthetic construct
  source 1..20: mol_type = other RNA
tctttccctcactgtggcag

SEQ ID NO: 16179 - RNA, 20 nt, synthetic construct
  source 1..20: mol_type = other RNA
cactgtggcaggggccgtgc

SEQ ID NO: 16180 - RNA, 20 nt, synthetic construct
  source 1..20: mol_type = other RNA
cacggcccctgccacagtga

SEQ ID NO: 16181 - RNA, 20 nt, synthetic construct
  source 1..20: mol_type = other RNA
gcacggcccctgccacagtg

SEQ ID NO: 16182 - RNA, 20 nt, synthetic construct
  source 1..20: mol_type = other RNA
tgtggcaggggccgtgcagg

SEQ ID NO: 16183 - RNA, 20 nt, synthetic construct
  source 1..20: mol_type = other RNA
ggggccgtgcaggtggataa

SEQ ID NO: 16184 - RNA, 20 nt, synthetic construct
  source 1..20: mol_type = other RNA
tcttcctttatccacctgca

SEQ ID NO: 16185 - RNA, 20 nt, synthetic construct
  source 1..20: mol_type = other RNA
ataaaggaagagctggtttc

SEQ ID NO: 16186 - RNA, 20 nt, synthetic construct
  source 1..20: mol_type = other RNA
acgctgttacagtcactctc

SEQ ID NO: 16187 - RNA, 20 nt, synthetic construct
  source 1..20: mol_type = other RNA
cgttgactcgaagctagaga

SEQ ID NO: 16188 - RNA, 20 nt, synthetic construct
  source 1..20: mol_type = other RNA
tgactcgaagctagagatgg

SEQ ID NO: 16189 - RNA, 20 nt, synthetic construct
  source 1..20: mol_type = other RNA
gactcgaagctagagatgga

SEQ ID NO: 16190 - RNA, 20 nt, synthetic construct
  source 1..20: mol_type = other RNA
actcgaagctagagatggag

SEQ ID NO: 16191 - RNA, 20 nt, synthetic construct
  source 1..20: mol_type = other RNA
ctcgaagctagagatggagg

SEQ ID NO: 16192 - RNA, 20 nt, synthetic construct
  source 1..20: mol_type = other RNA
gaagctagagatggaggggg

SEQ ID NO: 16193 - RNA, 20 nt, synthetic construct
  source 1..20: mol_type = other RNA
ggtggccgtctcttagacat

SEQ ID NO: 16194 - RNA, 20 nt, synthetic construct
  source 1..20: mol_type = other RNA
ggtgtccaatgtctaagaga

SEQ ID NO: 16195 - RNA, 20 nt, synthetic construct
  source 1..20: mol_type = other RNA
acacctctcagagcctcctg

SEQ ID NO: 16196 - RNA, 20 nt, synthetic construct
  source 1..20: mol_type = other RNA
cacctctcagagcctcctga

SEQ ID NO: 16197 - RNA, 20 nt, synthetic construct
  source 1..20: mol_type = other RNA
agccctcaggaggctctgag

SEQ ID NO: 16198 - RNA, 20 nt, synthetic construct
  source 1..20: mol_type = other RNA
aagacaaagaagccctcagg

SEQ ID NO: 16199 - RNA, 20 nt, synthetic construct
  source 1..20: mol_type = other RNA
tagaagacaaagaagccctc

SEQ ID NO: 16200 - RNA, 20 nt, synthetic construct
  source 1..20: mol_type = other RNA
ttgtcttctagaatctctac

SEQ ID NO: 16201 - RNA, 20 nt, synthetic construct
  source 1..20: mol_type = other RNA
tcttctagaatctctaccgg

SEQ ID NO: 16202 - RNA, 20 nt, synthetic construct
  source 1..20: mol_type = other RNA
tctaccggtggtcctcctgc

SEQ ID NO: 16203 - RNA, 20 nt, synthetic construct
  source 1..20: mol_type = other RNA
ggtggtcctcctgcaggttc

SEQ ID NO: 16204 - RNA, 20 nt, synthetic construct
  source 1..20: mol_type = other RNA
agaacctgcaggaggaccac

SEQ ID NO: 16205 - RNA, 20 nt, synthetic construct
  source 1..20: mol_type = other RNA
tgtgagccagaacctgcagg

SEQ ID NO: 16206 - RNA, 20 nt, synthetic construct
  source 1..20: mol_type = other RNA
gtctgtgagccagaacctgc

SEQ ID NO: 16207 - RNA, 20 nt, synthetic construct
  source 1..20: mol_type = other RNA
tgcctttttttccctccctg

SEQ ID NO: 16208 - RNA, 20 nt, synthetic construct
  source 1..20: mol_type = other RNA
cgcctcagggagggaaaaaa

SEQ ID NO: 16209 - RNA, 20 nt, synthetic construct
  source 1..20: mol_type = other RNA
tttccctccctgaggcgcct

SEQ ID NO: 16210 - RNA, 20 nt, synthetic construct
  source 1..20: mol_type = other RNA
ctgccaaggcgcctcaggga

SEQ ID NO: 16211 - RNA, 20 nt, synthetic construct
  source 1..20: mol_type = other RNA
tctgccaaggcgcctcaggg

SEQ ID NO: 16212 - RNA, 20 nt, synthetic construct
  source 1..20: mol_type = other RNA
tcttctgccaaggcgcctca

SEQ ID NO: 16213 - RNA, 20 nt, synthetic construct
  source 1..20: mol_type = other RNA
ctcttctgccaaggcgcctc

SEQ ID NO: 16214 - RNA, 20 nt, synthetic construct
  source 1..20: mol_type = other RNA
agggtcacgctcttctgcca

SEQ ID NO: 16215 - RNA, 20 nt, synthetic construct
  source 1..20: mol_type = other RNA
agagcgtgaccctgtgagcc

SEQ ID NO: 16216 - RNA, 20 nt, synthetic construct
  source 1..20: mol_type = other RNA
taaggggggcctggctcaca

SEQ ID NO: 16217 - RNA, 20 nt, synthetic construct
  source 1..20: mol_type = other RNA
ctaaggggggcctggctcac

SEQ ID NO: 16218 - RNA, 20 nt, synthetic construct
  source 1..20: mol_type = other RNA
aagcagagctaaggggggcc

SEQ ID NO: 16219 - RNA, 20 nt, synthetic construct
  source 1..20: mol_type = other RNA
atctgaagcagagctaaggg

SEQ ID NO: 16220 - RNA, 20 nt, synthetic construct
  source 1..20: mol_type = other RNA
gatctgaagcagagctaagg

SEQ ID NO: 16221 - RNA, 20 nt, synthetic construct
  source 1..20: mol_type = other RNA
tgatctgaagcagagctaag

SEQ ID NO: 16222 - RNA, 20 nt, synthetic construct
  source 1..20: mol_type = other RNA
gtgatctgaagcagagctaa

SEQ ID NO: 16223 - RNA, 20 nt, synthetic construct
  source 1..20: mol_type = other RNA
tgtgatctgaagcagagcta

SEQ ID NO: 16224 - RNA, 20 nt, synthetic construct
  source 1..20: mol_type = other RNA
cagacagactcgcgagttgc

SEQ ID NO: 16225 - RNA, 20 nt, synthetic construct
  source 1..20: mol_type = other RNA
cgcgagttgctggacctctt

SEQ ID NO: 16226 - RNA, 20 nt, synthetic construct
  source 1..20: mol_type = other RNA
tcaaacacttaataccaaag

SEQ ID NO: 16227 - RNA, 20 nt, synthetic construct
  source 1..20: mol_type = other RNA
gtattaagtgtttgaatcca

SEQ ID NO: 16228 - RNA, 20 nt, synthetic construct
  source 1..20: mol_type = other RNA
ttaagtgtttgaatccatgg

SEQ ID NO: 16229 - RNA, 20 nt, synthetic construct
  source 1..20: mol_type = other RNA
taagtgtttgaatccatggt

SEQ ID NO: 16230 - RNA, 20 nt, synthetic construct
  source 1..20: mol_type = other RNA
tacttgcaaaaggcccacca

SEQ ID NO: 16231 - RNA, 20 nt, synthetic construct
  source 1..20: mol_type = other RNA
gagctaacgctacttgcaaa

SEQ ID NO: 16232 - RNA, 20 nt, synthetic construct
  source 1..20: mol_type = other RNA
ttaaatgttgaactgagcta

SEQ ID NO: 16233 - RNA, 20 nt, synthetic construct
  source 1..20: mol_type = other RNA
gctaaggatgcactttcttg

SEQ ID NO: 16234 - RNA, 20 nt, synthetic construct
  source 1..20: mol_type = other RNA
cactttcttgtggacataga

SEQ ID NO: 16235 - RNA, 20 nt, synthetic construct
  source 1..20: mol_type = other RNA
actttcttgtggacatagaa

SEQ ID NO: 16236 - RNA, 20 nt, synthetic construct
  source 1..20: mol_type = other RNA
ctttcttgtggacatagaag

SEQ ID NO: 16237 - RNA, 20 nt, synthetic construct
  source 1..20: mol_type = other RNA
acatagaaggggcccacgta

SEQ ID NO: 16238 - RNA, 20 nt, synthetic construct
  source 1..20: mol_type = other RNA
gcccacgtaaggccctgagt

SEQ ID NO: 16239 - RNA, 20 nt, synthetic construct
  source 1..20: mol_type = other RNA
gcctactcagggccttacgt

SEQ ID NO: 16240 - RNA, 20 nt, synthetic construct
  source 1..20: mol_type = other RNA
agcctactcagggccttacg

SEQ ID NO: 16241 - RNA, 20 nt, synthetic construct
  source 1..20: mol_type = other RNA
gcaactaaggagcctactca

SEQ ID NO: 16242 - RNA, 20 nt, synthetic construct
  source 1..20: mol_type = other RNA
agcaactaaggagcctactc

SEQ ID NO: 16243 - RNA, 20 nt, synthetic construct
  source 1..20: mol_type = other RNA
agttgctgctttacctgatg

SEQ ID NO: 16244 - RNA, 20 nt, synthetic construct
  source 1..20: mol_type = other RNA
atcaggtaaagcagcaacta

SEQ ID NO: 16245 - RNA, 20 nt, synthetic construct
  source 1..20: mol_type = other RNA
taatctctttggccctcatc

SEQ ID NO: 16246 - RNA, 20 nt, synthetic construct
  source 1..20: mol_type = other RNA
cgaggcagagttaatctctt

SEQ ID NO: 16247 - RNA, 20 nt, synthetic construct
  source 1..20: mol_type = other RNA
ttttctgagacatggcaacg

SEQ ID NO: 16248 - RNA, 20 nt, synthetic construct
  source 1..20: mol_type = other RNA
atggcaacttttctgagaca

SEQ ID NO: 16249 - RNA, 20 nt, synthetic construct
  source 1..20: mol_type = other RNA
gttgccatatttcacccaga

SEQ ID NO: 16250 - RNA, 20 nt, synthetic construct
  source 1..20: mol_type = other RNA
ttgccatatttcacccagaa

SEQ ID NO: 16251 - RNA, 20 nt, synthetic construct
  source 1..20: mol_type = other RNA
tgccatatttcacccagaag

SEQ ID NO: 16252 - RNA, 20 nt, synthetic construct
  source 1..20: mol_type = other RNA
agccccttctgggtgaaata

SEQ ID NO: 16253 - RNA, 20 nt, synthetic construct
  source 1..20: mol_type = other RNA
gaggaaaacaagccccttct

SEQ ID NO: 16254 - RNA, 20 nt, synthetic construct
  source 1..20: mol_type = other RNA
agaggaaaacaagccccttc

SEQ ID NO: 16255 - RNA, 20 nt, synthetic construct
  source 1..20: mol_type = other RNA
atggttaaagtaagagtaag

SEQ ID NO: 16256 - RNA, 20 nt, synthetic construct
  source 1..20: mol_type = other RNA
tcttactttaaccatgtgcc

SEQ ID NO: 16257 - RNA, 20 nt, synthetic construct
  source 1..20: mol_type = other RNA
tactttaaccatgtgcctgg

SEQ ID NO: 16258 - RNA, 20 nt, synthetic construct
  source 1..20: mol_type = other RNA
tgtgcctggaggagccattc

SEQ ID NO: 16259 - RNA, 20 nt, synthetic construct
  source 1..20: mol_type = other RNA
gtgcctggaggagccattct

SEQ ID NO: 16260 - RNA, 20 nt, synthetic construct
  source 1..20: mol_type = other RNA
gaatggctcctccaggcaca

SEQ ID NO: 16261 - RNA, 20 nt, synthetic construct
  source 1..20: mol_type = other RNA
gagcccagaatggctcctcc

SEQ ID NO: 16262 - RNA, 20 nt, synthetic construct
  source 1..20: mol_type = other RNA
gcaagtgcaagagcccagaa

SEQ ID NO: 16263 - RNA, 20 nt, synthetic construct
  source 1..20: mol_type = other RNA
ttgcccagcctttctttgcc

SEQ ID NO: 16264 - RNA, 20 nt, synthetic construct
  source 1..20: mol_type = other RNA
tgcccagcctttctttgcca

SEQ ID NO: 16265 - RNA, 20 nt, synthetic construct
  source 1..20: mol_type = other RNA
gcccagcctttctttgccag

SEQ ID NO: 16266 - RNA, 20 nt, synthetic construct
  source 1..20: mol_type = other RNA
gcccctggcaaagaaaggct

SEQ ID NO: 16267 - RNA, 20 nt, synthetic construct
  source 1..20: mol_type = other RNA
tgcccctggcaaagaaaggc

SEQ ID NO: 16268 - RNA, 20 nt, synthetic construct
  source 1..20: mol_type = other RNA
ttctttgccaggggcagaga

SEQ ID NO: 16269 - RNA, 20 nt, synthetic construct
  source 1..20: mol_type = other RNA
tctttgccaggggcagagaa

SEQ ID NO: 16270 - RNA, 20 nt, synthetic construct
  source 1..20: mol_type = other RNA
tctctgcccctggcaaagaa

SEQ ID NO: 16271 - RNA, 20 nt, synthetic construct
  source 1..20: mol_type = other RNA
gccaggggcagagaagggaa

SEQ ID NO: 16272 - RNA, 20 nt, synthetic construct
  source 1..20: mol_type = other RNA
ccaggggcagagaagggaaa

SEQ ID NO: 16273 - RNA, 20 nt, synthetic construct
  source 1..20: mol_type = other RNA
caggggcagagaagggaaag

SEQ ID NO: 16274 - RNA, 20 nt, synthetic construct
  source 1..20: mol_type = other RNA
aggggcagagaagggaaagg

SEQ ID NO: 16275 - RNA, 20 nt, synthetic construct
  source 1..20: mol_type = other RNA
ccctttcccttctctgcccc

SEQ ID NO: 16276 - RNA, 20 nt, synthetic construct
  source 1..20: mol_type = other RNA
ggggtagattgagtgtgcca

SEQ ID NO: 16277 - RNA, 20 nt, synthetic construct
  source 1..20: mol_type = other RNA
gggtagattgagtgtgccaa

SEQ ID NO: 16278 - RNA, 20 nt, synthetic construct
  source 1..20: mol_type = other RNA
agtgtgccaagggccgtgca

SEQ ID NO: 16279 - RNA, 20 nt, synthetic construct
  source 1..20: mol_type = other RNA
gtgtgccaagggccgtgcaa

SEQ ID NO: 16280 - RNA, 20 nt, synthetic construct
  source 1..20: mol_type = other RNA
gccaagggccgtgcaagggc

SEQ ID NO: 16281 - RNA, 20 nt, synthetic construct
  source 1..20: mol_type = other RNA
gcctgcccttgcacggccct

SEQ ID NO: 16282 - RNA, 20 nt, synthetic construct
  source 1..20: mol_type = other RNA
aaagcaagcctgcccttgca

SEQ ID NO: 16283 - RNA, 20 nt, synthetic construct
  source 1..20: mol_type = other RNA
tgctttccacccatctgctg

SEQ ID NO: 16284 - RNA, 20 nt, synthetic construct
  source 1..20: mol_type = other RNA
gctttccacccatctgctga

SEQ ID NO: 16285 - RNA, 20 nt, synthetic construct
  source 1..20: mol_type = other RNA
gggctccctcagcagatggg

SEQ ID NO: 16286 - RNA, 20 nt, synthetic construct
  source 1..20: mol_type = other RNA
agagggctccctcagcagat

SEQ ID NO: 16287 - RNA, 20 nt, synthetic construct
  source 1..20: mol_type = other RNA
gagagggctccctcagcaga

SEQ ID NO: 16288 - RNA, 20 nt, synthetic construct
  source 1..20: mol_type = other RNA
aggcaaggagcgagaggaga

SEQ ID NO: 16289 - RNA, 20 nt, synthetic construct
  source 1..20: mol_type = other RNA
gaggcaaggagcgagaggag

SEQ ID NO: 16290 - RNA, 20 nt, synthetic construct
  source 1..20: mol_type = other RNA
gaacagaggcaaggagcgag

SEQ ID NO: 16291 - RNA, 20 nt, synthetic construct
  source 1..20: mol_type = other RNA
aacaggtgtgaacagaggca

SEQ ID NO: 16292 - RNA, 20 nt, synthetic construct
  source 1..20: mol_type = other RNA
tctgttcacacctgttgtct

SEQ ID NO: 16293 - RNA, 20 nt, synthetic construct
  source 1..20: mol_type = other RNA
aagacaacaggtgtgaacag

SEQ ID NO: 16294 - RNA, 20 nt, synthetic construct
  source 1..20: mol_type = other RNA
cacacctgttgtcttggaag

SEQ ID NO: 16295 - RNA, 20 nt, synthetic construct
  source 1..20: mol_type = other RNA
cctgttgtcttggaagagga

SEQ ID NO: 16296 - RNA, 20 nt, synthetic construct
  source 1..20: mol_type = other RNA
ccatcctcttccaagacaac

SEQ ID NO: 16297 - RNA, 20 nt, synthetic construct
  source 1..20: mol_type = other RNA
aggatggtccctttgtctta

SEQ ID NO: 16298 - RNA, 20 nt, synthetic construct
  source 1..20: mol_type = other RNA
tcacaaagccttaagacaaa

SEQ ID NO: 16299 - RNA, 20 nt, synthetic construct
  source 1..20: mol_type = other RNA
atcacaaagccttaagacaa

SEQ ID NO: 16300 - RNA, 20 nt, synthetic construct
  source 1..20: mol_type = other RNA
tgataaagtcatctccagtt

SEQ ID NO: 16301 - RNA, 20 nt, synthetic construct
  source 1..20: mol_type = other RNA
aaacaggtgcagatcctaac

SEQ ID NO: 16302 - RNA, 20 nt, synthetic construct
  source 1..20: mol_type = other RNA
gtttccttcgtaatagtgcc

SEQ ID NO: 16303 - RNA, 20 nt, synthetic construct
  source 1..20: mol_type = other RNA
ggcactattacgaaggaaac

SEQ ID NO: 16304 - RNA, 20 nt, synthetic construct
  source 1..20: mol_type = other RNA
tccttcgtaatagtgcctgg

SEQ ID NO: 16305 - RNA, 20 nt, synthetic construct
  source 1..20: mol_type = other RNA
gccgccaggcactattacga

SEQ ID NO: 16306 - RNA, 20 nt, synthetic construct
  source 1..20: mol_type = other RNA
ggcggcctttctgaagttac

SEQ ID NO: 16307 - RNA, 20 nt, synthetic construct
  source 1..20: mol_type = other RNA
gtaacttcagaaaggccgcc

SEQ ID NO: 16308 - RNA, 20 nt, synthetic construct
  source 1..20: mol_type = other RNA
ggcctttctgaagttacagg

SEQ ID NO: 16309 - RNA, 20 nt, synthetic construct
  source 1..20: mol_type = other RNA
tttctgaagttacaggtggt

SEQ ID NO: 16310 - RNA, 20 nt, synthetic construct
  source 1..20: mol_type = other RNA
ttctgaagttacaggtggtt

SEQ ID NO: 16311 - RNA, 20 nt, synthetic construct
  source 1..20: mol_type = other RNA
aaccacctgtaacttcagaa

SEQ ID NO: 16312 - RNA, 20 nt, synthetic construct
  source 1..20: mol_type = other RNA
cctctcgcatgcagaacatc

SEQ ID NO: 16313 - RNA, 20 nt, synthetic construct
  source 1..20: mol_type = other RNA
cagatgttctgcatgcgaga

SEQ ID NO: 16314 - RNA, 20 nt, synthetic construct
  source 1..20: mol_type = other RNA
ccagatgttctgcatgcgag

SEQ ID NO: 16315 - RNA, 20 nt, synthetic construct
  source 1..20: mol_type = other RNA
atctggtagattgatctgcc

SEQ ID NO: 16316 - RNA, 20 nt, synthetic construct
  source 1..20: mol_type = other RNA
ggtagattgatctgccaggc

SEQ ID NO: 16317 - RNA, 20 nt, synthetic construct
  source 1..20: mol_type = other RNA
gtagattgatctgccaggct

SEQ ID NO: 16318 - RNA, 20 nt, synthetic construct
  source 1..20: mol_type = other RNA
gattgatctgccaggctggg

SEQ ID NO: 16319 - RNA, 20 nt, synthetic construct
  source 1..20: mol_type = other RNA
agcagtagaaccacccagcc

SEQ ID NO: 16320 - RNA, 20 nt, synthetic construct
  source 1..20: mol_type = other RNA
aactctttaagaaaaaaaaa

SEQ ID NO: 16321 - RNA, 20 nt, synthetic construct
  source 1..20: mol_type = other RNA
gtaagtaccatgtttccttg

SEQ ID NO: 16322 - RNA, 20 nt, synthetic construct
  source 1..20: mol_type = other RNA
gcatacaccacaaggaaaca

SEQ ID NO: 16323 - RNA, 20 nt, synthetic construct
  source 1..20: mol_type = other RNA
ttgtggtgtatgctctgttc

SEQ ID NO: 16324 - RNA, 20 nt, synthetic construct
  source 1..20: mol_type = other RNA
agaacagagcatacaccaca

SEQ ID NO: 16325 - RNA, 20 nt, synthetic construct
  source 1..20: mol_type = other RNA
tttcaaatcaaatgcctgtt

SEQ ID NO: 16326 - RNA, 20 nt, synthetic construct
  source 1..20: mol_type = other RNA
ttcaaatcaaatgcctgttt

SEQ ID NO: 16327 - RNA, 20 nt, synthetic construct
  source 1..20: mol_type = other RNA
aaatcaaatgcctgtttggg

SEQ ID NO: 16328 - RNA, 20 nt, synthetic construct
  source 1..20: mol_type = other RNA
acgttcatctcctcccaaac

SEQ ID NO: 16329 - RNA, 20 nt, synthetic construct
  source 1..20: mol_type = other RNA
gtctattagatttgcactgc

SEQ ID NO: 16330 - RNA, 20 nt, synthetic construct
  source 1..20: mol_type = other RNA
aacaataagacagctattca

SEQ ID NO: 16331 - RNA, 20 nt, synthetic construct
  source 1..20: mol_type = other RNA
aatcgattgactaatcttac

SEQ ID NO: 16332 - RNA, 20 nt, synthetic construct
  source 1..20: mol_type = other RNA
ttggactcactcaagtaaac

SEQ ID NO: 16333 - RNA, 20 nt, synthetic construct
  source 1..20: mol_type = other RNA
tggactcactcaagtaaaca

SEQ ID NO: 16334 - RNA, 20 nt, synthetic construct
  source 1..20: mol_type = other RNA
ggactcactcaagtaaacag

SEQ ID NO: 16335 - RNA, 20 nt, synthetic construct
  source 1..20: mol_type = other RNA
caagtaaacaggggctttat

SEQ ID NO: 16336 - RNA, 20 nt, synthetic construct
  source 1..20: mol_type = other RNA
gctttattggcttatagacc

SEQ ID NO: 16337 - RNA, 20 nt, synthetic construct
  source 1..20: mol_type = other RNA
ctttattggcttatagacct

SEQ ID NO: 16338 - RNA, 20 nt, synthetic construct
  source 1..20: mol_type = other RNA
cttatagacctgggcagtcc

SEQ ID NO: 16339 - RNA, 20 nt, synthetic construct
  source 1..20: mol_type = other RNA
gggcagtccaggtgtagatc

SEQ ID NO: 16340 - RNA, 20 nt, synthetic construct
  source 1..20: mol_type = other RNA
gatctacacctggactgccc

SEQ ID NO: 16341 - RNA, 20 nt, synthetic construct
  source 1..20: mol_type = other RNA
tgtagatctggttccagaca

SEQ ID NO: 16342 - RNA, 20 nt, synthetic construct
  source 1..20: mol_type = other RNA
gtctctgaatcagccttgtc

SEQ ID NO: 16343 - RNA, 20 nt, synthetic construct
  source 1..20: mol_type = other RNA
gctgattcagagactccacg

SEQ ID NO: 16344 - RNA, 20 nt, synthetic construct
  source 1..20: mol_type = other RNA
tcagagactccacgtggtca

SEQ ID NO: 16345 - RNA, 20 nt, synthetic construct
  source 1..20: mol_type = other RNA
acaacagagccttgaccacg

SEQ ID NO: 16346 - RNA, 20 nt, synthetic construct
  source 1..20: mol_type = other RNA
tctgttgtttgtcaatccct

SEQ ID NO: 16347 - RNA, 20 nt, synthetic construct
  source 1..20: mol_type = other RNA
tggctcctccacttccagtt

SEQ ID NO: 16348 - RNA, 20 nt, synthetic construct
  source 1..20: mol_type = other RNA
actggaagtggaggagccaa

SEQ ID NO: 16349 - RNA, 20 nt, synthetic construct
  source 1..20: mol_type = other RNA
aactggaagtggaggagcca

SEQ ID NO: 16350 - RNA, 20 nt, synthetic construct
  source 1..20: mol_type = other RNA
agaagccaaactggaagtgg

SEQ ID NO: 16351 - RNA, 20 nt, synthetic construct
  source 1..20: mol_type = other RNA
gacagaagccaaactggaag

SEQ ID NO: 16352 - RNA, 20 nt, synthetic construct
  source 1..20: mol_type = other RNA
tgtgaggacagaagccaaac

SEQ ID NO: 16353 - RNA, 20 nt, synthetic construct
  source 1..20: mol_type = other RNA
cctcacagtctctctccatg

SEQ ID NO: 16354 - RNA, 20 nt, synthetic construct
  source 1..20: mol_type = other RNA
ccacatggagagagactgtg

SEQ ID NO: 16355 - RNA, 20 nt, synthetic construct
  source 1..20: mol_type = other RNA
tctccatgtggcaaacaaga

SEQ ID NO: 16356 - RNA, 20 nt, synthetic construct
  source 1..20: mol_type = other RNA
gtggcaaacaagatggctac

SEQ ID NO: 16357 - RNA, 20 nt, synthetic construct
  source 1..20: mol_type = other RNA
tagccatcttgtttgccaca

SEQ ID NO: 16358 - RNA, 20 nt, synthetic construct
  source 1..20: mol_type = other RNA
gcaaacaagatggctactgg

SEQ ID NO: 16359 - RNA, 20 nt, synthetic construct
  source 1..20: mol_type = other RNA
agatggctactggtggtccc

SEQ ID NO: 16360 - RNA, 20 nt, synthetic construct
  source 1..20: mol_type = other RNA
aggttcacgtcctctcagct

SEQ ID NO: 16361 - RNA, 20 nt, synthetic construct
  source 1..20: mol_type = other RNA
agctgagaggacgtgaacct

SEQ ID NO: 16362 - RNA, 20 nt, synthetic construct
  source 1..20: mol_type = other RNA
aagctgagaggacgtgaacc

SEQ ID NO: 16363 - RNA, 20 nt, synthetic construct
  source 1..20: mol_type = other RNA
tgctggatttccaagctgag

SEQ ID NO: 16364 - RNA, 20 nt, synthetic construct
  source 1..20: mol_type = other RNA
gtgagacatcttcttgctgc

SEQ ID NO: 16365 - RNA, 20 nt, synthetic construct
  source 1..20: mol_type = other RNA
aaagtccataactcaatcct

SEQ ID NO: 16366 - RNA, 20 nt, synthetic construct
  source 1..20: mol_type = other RNA
aagtccataactcaatcctt

SEQ ID NO: 16367 - RNA, 20 nt, synthetic construct
  source 1..20: mol_type = other RNA
aggattgagttatggacttt

SEQ ID NO: 16368 - RNA, 20 nt, synthetic construct
  source 1..20: mol_type = other RNA
aaggattgagttatggactt

SEQ ID NO: 16369 - RNA, 20 nt, synthetic construct
  source 1..20: mol_type = other RNA
tcttcccaaggattgagtta

SEQ ID NO: 16370 - RNA, 20 nt, synthetic construct
  source 1..20: mol_type = other RNA
atccttgggaagactgtagt

SEQ ID NO: 16371 - RNA, 20 nt, synthetic construct
  source 1..20: mol_type = other RNA
gaccaactacagtcttccca

SEQ ID NO: 16372 - RNA, 20 nt, synthetic construct
  source 1..20: mol_type = other RNA
agactgtagttggtcctgct

SEQ ID NO: 16373 - RNA, 20 nt, synthetic construct
  source 1..20: mol_type = other RNA
gatagttacgtgttcctagc

SEQ ID NO: 16374 - RNA, 20 nt, synthetic construct
  source 1..20: mol_type = other RNA
tatccaactatcctccagat

SEQ ID NO: 16375 - RNA, 20 nt, synthetic construct
  source 1..20: mol_type = other RNA
atccaactatcctccagata

SEQ ID NO: 16376 - RNA, 20 nt, synthetic construct
  source 1..20: mol_type = other RNA
ctatcctccagatagggagc

SEQ ID NO: 16377 - RNA, 20 nt, synthetic construct
  source 1..20: mol_type = other RNA
tatcctccagatagggagct

SEQ ID NO: 16378 - RNA, 20 nt, synthetic construct
  source 1..20: mol_type = other RNA
atcctccagatagggagctg

SEQ ID NO: 16379 - RNA, 20 nt, synthetic construct
  source 1..20: mol_type = other RNA
cagatagggagctggggaga

SEQ ID NO: 16380 - RNA, 20 nt, synthetic construct
  source 1..20: mol_type = other RNA
agatagggagctggggagat

SEQ ID NO: 16381 - RNA, 20 nt, synthetic construct
  source 1..20: mol_type = other RNA
catctccccagctccctatc

SEQ ID NO: 16382 - RNA, 20 nt, synthetic construct
  source 1..20: mol_type = other RNA
ggagctggggagatgggaga

SEQ ID NO: 16383 - RNA, 20 nt, synthetic construct
  source 1..20: mol_type = other RNA
gagctggggagatgggagat

SEQ ID NO: 16384 - RNA, 20 nt, synthetic construct
  source 1..20: mol_type = other RNA
gggagatgggctcctctgac

SEQ ID NO: 16385 - RNA, 20 nt, synthetic construct
  source 1..20: mol_type = other RNA
tcctctgacaggacaccctg

SEQ ID NO: 16386 - RNA, 20 nt, synthetic construct
  source 1..20: mol_type = other RNA
accacagggtgtcctgtcag

SEQ ID NO: 16387 - RNA, 20 nt, synthetic construct
  source 1..20: mol_type = other RNA
gtggttcacgtccactcttg

SEQ ID NO: 16388 - RNA, 20 nt, synthetic construct
  source 1..20: mol_type = other RNA
aagagtggacgtgaaccaca

SEQ ID NO: 16389 - RNA, 20 nt, synthetic construct
  source 1..20: mol_type = other RNA
caagagtggacgtgaaccac

SEQ ID NO: 16390 - RNA, 20 nt, synthetic construct
  source 1..20: mol_type = other RNA
tcacgtccactcttgtggcc

SEQ ID NO: 16391 - RNA, 20 nt, synthetic construct
  source 1..20: mol_type = other RNA
cacgtccactcttgtggcct

SEQ ID NO: 16392 - RNA, 20 nt, synthetic construct
  source 1..20: mol_type = other RNA
ctcttgtggcctgggtatat

SEQ ID NO: 16393 - RNA, 20 nt, synthetic construct
  source 1..20: mol_type = other RNA
tcttgtggcctgggtatatt

SEQ ID NO: 16394 - RNA, 20 nt, synthetic construct
  source 1..20: mol_type = other RNA
atatacccaggccacaagag

SEQ ID NO: 16395 - RNA, 20 nt, synthetic construct
  source 1..20: mol_type = other RNA
gcctgggtatattgggaatg

SEQ ID NO: 16396 - RNA, 20 nt, synthetic construct
  source 1..20: mol_type = other RNA
cctgggtatattgggaatgc

SEQ ID NO: 16397 - RNA, 20 nt, synthetic construct
  source 1..20: mol_type = other RNA
ctgggtatattgggaatgcg

SEQ ID NO: 16398 - RNA, 20 nt, synthetic construct
  source 1..20: mol_type = other RNA
cccgcattcccaatataccc

SEQ ID NO: 16399 - RNA, 20 nt, synthetic construct
  source 1..20: mol_type = other RNA
aaagaattcacagccccaca

SEQ ID NO: 16400 - RNA, 20 nt, synthetic construct
  source 1..20: mol_type = other RNA
acagccccacaaggttcgtg

SEQ ID NO: 16401 - RNA, 20 nt, synthetic construct
  source 1..20: mol_type = other RNA
ccacaaggttcgtgtggaaa

SEQ ID NO: 16402 - RNA, 20 nt, synthetic construct
  source 1..20: mol_type = other RNA
cacaaggttcgtgtggaaaa

SEQ ID NO: 16403 - RNA, 20 nt, synthetic construct
  source 1..20: mol_type = other RNA
acaaggttcgtgtggaaaag

SEQ ID NO: 16404 - RNA, 20 nt, synthetic construct
  source 1..20: mol_type = other RNA
ttttccacacgaaccttgtg

SEQ ID NO: 16405 - RNA, 20 nt, synthetic construct
  source 1..20: mol_type = other RNA
cttttccacacgaaccttgt

SEQ ID NO: 16406 - RNA, 20 nt, synthetic construct
  source 1..20: mol_type = other RNA
aggttcgtgtggaaaagggg

SEQ ID NO: 16407 - RNA, 20 nt, synthetic construct
  source 1..20: mol_type = other RNA
cttaattttatggctcttct

SEQ ID NO: 16408 - RNA, 20 nt, synthetic construct
  source 1..20: mol_type = other RNA
tcttaattttatggctcttc

SEQ ID NO: 16409 - RNA, 20 nt, synthetic construct
  source 1..20: mol_type = other RNA
gcagtgctttcttaatttta

SEQ ID NO: 16410 - RNA, 20 nt, synthetic construct
  source 1..20: mol_type = other RNA
aaaccagtcatttaagttct

SEQ ID NO: 16411 - RNA, 20 nt, synthetic construct
  source 1..20: mol_type = other RNA
ctgccaagaacttaaatgac

SEQ ID NO: 16412 - RNA, 20 nt, synthetic construct
  source 1..20: mol_type = other RNA
cctagtgcttcattttgctc

SEQ ID NO: 16413 - RNA, 20 nt, synthetic construct
  source 1..20: mol_type = other RNA
ccagagcaaaatgaagcact

SEQ ID NO: 16414 - RNA, 20 nt, synthetic construct
  source 1..20: mol_type = other RNA
aaaaagcagatctgctctgc

SEQ ID NO: 16415 - RNA, 20 nt, synthetic construct
  source 1..20: mol_type = other RNA
aaaagcagatctgctctgct

SEQ ID NO: 16416 - RNA, 20 nt, synthetic construct
  source 1..20: mol_type = other RNA
aaagcagatctgctctgctg

SEQ ID NO: 16417 - RNA, 20 nt, synthetic construct
  source 1..20: mol_type = other RNA
ctctgctggggcaattctaa

SEQ ID NO: 16418 - RNA, 20 nt, synthetic construct
  source 1..20: mol_type = other RNA
tccagtgtgctttgagaaag

SEQ ID NO: 16419 - RNA, 20 nt, synthetic construct
  source 1..20: mol_type = other RNA
tttctcaaagcacactggaa

SEQ ID NO: 16420 - RNA, 20 nt, synthetic construct
  source 1..20: mol_type = other RNA
agtgtgctttgagaaagtgg

SEQ ID NO: 16421 - RNA, 20 nt, synthetic construct
  source 1..20: mol_type = other RNA
gtgtgctttgagaaagtgga

SEQ ID NO: 16422 - RNA, 20 nt, synthetic construct
  source 1..20: mol_type = other RNA
tccactttctcaaagcacac

SEQ ID NO: 16423 - RNA, 20 nt, synthetic construct
  source 1..20: mol_type = other RNA
gagaaagtggagggactgcg

SEQ ID NO: 16424 - RNA, 20 nt, synthetic construct
  source 1..20: mol_type = other RNA
gagggactgcgtggtattgc

SEQ ID NO: 16425 - RNA, 20 nt, synthetic construct
  source 1..20: mol_type = other RNA
agggactgcgtggtattgct

SEQ ID NO: 16426 - RNA, 20 nt, synthetic construct
  source 1..20: mol_type = other RNA
attgctgggcttcccatttc

SEQ ID NO: 16427 - RNA, 20 nt, synthetic construct
  source 1..20: mol_type = other RNA
gcttcccatttcaggagacc

SEQ ID NO: 16428 - RNA, 20 nt, synthetic construct
  source 1..20: mol_type = other RNA
cttcccatttcaggagacct

SEQ ID NO: 16429 - RNA, 20 nt, synthetic construct
  source 1..20: mol_type = other RNA
gggcccaggtctcctgaaat

SEQ ID NO: 16430 - RNA, 20 nt, synthetic construct
  source 1..20: mol_type = other RNA
tgggcccaggtctcctgaaa

SEQ ID NO: 16431 - RNA, 20 nt, synthetic construct
  source 1..20: mol_type = other RNA
gtcatagaactgctgggccc

SEQ ID NO: 16432 - RNA, 20 nt, synthetic construct
  source 1..20: mol_type = other RNA
catcatgtcatagaactgct

SEQ ID NO: 16433 - RNA, 20 nt, synthetic construct
  source 1..20: mol_type = other RNA
tcatcatgtcatagaactgc

SEQ ID NO: 16434 - RNA, 20 nt, synthetic construct
  source 1..20: mol_type = other RNA
tgacatgatgatgagcactc

SEQ ID NO: 16435 - RNA, 20 nt, synthetic construct
  source 1..20: mol_type = other RNA
ctggacccaaaccagacacc

SEQ ID NO: 16436 - RNA, 20 nt, synthetic construct
  source 1..20: mol_type = other RNA
actggccaggtgtctggttt

SEQ ID NO: 16437 - RNA, 20 nt, synthetic construct
  source 1..20: mol_type = other RNA
cactggccaggtgtctggtt

SEQ ID NO: 16438 - RNA, 20 nt, synthetic construct
  source 1..20: mol_type = other RNA
caggacactggccaggtgtc

SEQ ID NO: 16439 - RNA, 20 nt, synthetic construct
  source 1..20: mol_type = other RNA
tcagaatcaggacactggcc

SEQ ID NO: 16440 - RNA, 20 nt, synthetic construct
  source 1..20: mol_type = other RNA
cagtctcagaatcaggacac

SEQ ID NO: 16441 - RNA, 20 nt, synthetic construct
  source 1..20: mol_type = other RNA
ggctcttcagtctcagaatc

SEQ ID NO: 16442 - RNA, 20 nt, synthetic construct
  source 1..20: mol_type = other RNA
actgaagagccctgtgaatg

SEQ ID NO: 16443 - RNA, 20 nt, synthetic construct
  source 1..20: mol_type = other RNA
ctgaagagccctgtgaatgt

SEQ ID NO: 16444 - RNA, 20 nt, synthetic construct
  source 1..20: mol_type = other RNA
gggcattgcccacattcaca

SEQ ID NO: 16445 - RNA, 20 nt, synthetic construct
  source 1..20: mol_type = other RNA
agggcattgcccacattcac

SEQ ID NO: 16446 - RNA, 20 nt, synthetic construct
  source 1..20: mol_type = other RNA
ggcaatgccctcctgctttc

SEQ ID NO: 16447 - RNA, 20 nt, synthetic construct
  source 1..20: mol_type = other RNA
gcaatgccctcctgctttct

SEQ ID NO: 16448 - RNA, 20 nt, synthetic construct
  source 1..20: mol_type = other RNA
caatgccctcctgctttctg

SEQ ID NO: 16449 - RNA, 20 nt, synthetic construct
  source 1..20: mol_type = other RNA
aatgccctcctgctttctgg

SEQ ID NO: 16450 - RNA, 20 nt, synthetic construct
  source 1..20: mol_type = other RNA
ctcctgctttctgggggtca

SEQ ID NO: 16451 - RNA, 20 nt, synthetic construct
  source 1..20: mol_type = other RNA
tcctgctttctgggggtcat

SEQ ID NO: 16452 - RNA, 20 nt, synthetic construct
  source 1..20: mol_type = other RNA
atgacccccagaaagcagga

SEQ ID NO: 16453 - RNA, 20 nt, synthetic construct
  source 1..20: mol_type = other RNA
catgacccccagaaagcagg

SEQ ID NO: 16454 - RNA, 20 nt, synthetic construct
  source 1..20: mol_type = other RNA
gctttctgggggtcatgggt

SEQ ID NO: 16455 - RNA, 20 nt, synthetic construct
  source 1..20: mol_type = other RNA
ctttctgggggtcatgggtg

SEQ ID NO: 16456 - RNA, 20 nt, synthetic construct
  source 1..20: mol_type = other RNA
acccatgacccccagaaagc

SEQ ID NO: 16457 - RNA, 20 nt, synthetic construct
  source 1..20: mol_type = other RNA
tcataaggcaagagctgaga

SEQ ID NO: 16458 - RNA, 20 nt, synthetic construct
  source 1..20: mol_type = other RNA
gatgttataaaaaactcata

SEQ ID NO: 16459 - RNA, 20 nt, synthetic construct
  source 1..20: mol_type = other RNA
ataacatcatttctcctttc

SEQ ID NO: 16460 - RNA, 20 nt, synthetic construct
  source 1..20: mol_type = other RNA
taacatcatttctcctttct

SEQ ID NO: 16461 - RNA, 20 nt, synthetic construct
  source 1..20: mol_type = other RNA
gagaaaactaacacccagaa

SEQ ID NO: 16462 - RNA, 20 nt, synthetic construct
  source 1..20: mol_type = other RNA
ttagttttctcatctatgtg

SEQ ID NO: 16463 - RNA, 20 nt, synthetic construct
  source 1..20: mol_type = other RNA
atttcaagttggacagatct

SEQ ID NO: 16464 - RNA, 20 nt, synthetic construct
  source 1..20: mol_type = other RNA
ttttcatttttatttcaagt

SEQ ID NO: 16465 - RNA, 20 nt, synthetic construct
  source 1..20: mol_type = other RNA
acctcaaattctgattcttt

SEQ ID NO: 16466 - RNA, 20 nt, synthetic construct
  source 1..20: mol_type = other RNA
tccaaaagaatcagaatttg

SEQ ID NO: 16467 - RNA, 20 nt, synthetic construct
  source 1..20: mol_type = other RNA
tcgttaactatgctgggaaa

SEQ ID NO: 16468 - RNA, 20 nt, synthetic construct
  source 1..20: mol_type = other RNA
gggagctcgttaactatgct

SEQ ID NO: 16469 - RNA, 20 nt, synthetic construct
  source 1..20: mol_type = other RNA
tgggagctcgttaactatgc

SEQ ID NO: 16470 - RNA, 20 nt, synthetic construct
  source 1..20: mol_type = other RNA
ggaggtaaagtgtctggtct

SEQ ID NO: 16471 - RNA, 20 nt, synthetic construct
  source 1..20: mol_type = other RNA
tggaggtaaagtgtctggtc

SEQ ID NO: 16472 - RNA, 20 nt, synthetic construct
  source 1..20: mol_type = other RNA
gacactttacctccattctc

SEQ ID NO: 16473 - RNA, 20 nt, synthetic construct
  source 1..20: mol_type = other RNA
gagaatggaggtaaagtgtc

SEQ ID NO: 16474 - RNA, 20 nt, synthetic construct
  source 1..20: mol_type = other RNA
acctccattctcaggcgctg

SEQ ID NO: 16475 - RNA, 20 nt, synthetic construct
  source 1..20: mol_type = other RNA
tccattctcaggcgctgagg

SEQ ID NO: 16476 - RNA, 20 nt, synthetic construct
  source 1..20: mol_type = other RNA
ccattctcaggcgctgagga

SEQ ID NO: 16477 - RNA, 20 nt, synthetic construct
  source 1..20: mol_type = other RNA
tcctcagcgcctgagaatgg

SEQ ID NO: 16478 - RNA, 20 nt, synthetic construct
  source 1..20: mol_type = other RNA
ttctcaggcgctgaggaggg

SEQ ID NO: 16479 - RNA, 20 nt, synthetic construct
  source 1..20: mol_type = other RNA
ccctcctcagcgcctgagaa

SEQ ID NO: 16480 - RNA, 20 nt, synthetic construct
  source 1..20: mol_type = other RNA
ggcgctgaggagggtggagc

SEQ ID NO: 16481 - RNA, 20 nt, synthetic construct
  source 1..20: mol_type = other RNA
agcaggcctgcaatgcatat

SEQ ID NO: 16482 - RNA, 20 nt, synthetic construct
  source 1..20: mol_type = other RNA
gcaggcctgcaatgcatata

SEQ ID NO: 16483 - RNA, 20 nt, synthetic construct
  source 1..20: mol_type = other RNA
caggcctgcaatgcatatag

SEQ ID NO: 16484 - RNA, 20 nt, synthetic construct
  source 1..20: mol_type = other RNA
caatgcatataggggaacaa

SEQ ID NO: 16485 - RNA, 20 nt, synthetic construct
  source 1..20: mol_type = other RNA
tgttcccctatatgcattgc

SEQ ID NO: 16486 - RNA, 20 nt, synthetic construct
  source 1..20: mol_type = other RNA
aaggcccagagacagagacg

SEQ ID NO: 16487 - RNA, 20 nt, synthetic construct
  source 1..20: mol_type = other RNA
aggcccagagacagagacgt

SEQ ID NO: 16488 - RNA, 20 nt, synthetic construct
  source 1..20: mol_type = other RNA
gttcccacgtctctgtctct

SEQ ID NO: 16489 - RNA, 20 nt, synthetic construct
  source 1..20: mol_type = other RNA
ggttcccacgtctctgtctc

SEQ ID NO: 16490 - RNA, 20 nt, synthetic construct
  source 1..20: mol_type = other RNA
aaccatgcagtgtaaaaaag

SEQ ID NO: 16491 - RNA, 20 nt, synthetic construct
  source 1..20: mol_type = other RNA
accatgcagtgtaaaaaagc

SEQ ID NO: 16492 - RNA, 20 nt, synthetic construct
  source 1..20: mol_type = other RNA
atgcagtgtaaaaaagcggg

SEQ ID NO: 16493 - RNA, 20 nt, synthetic construct
  source 1..20: mol_type = other RNA
tcccgcttttttacactgca

SEQ ID NO: 16494 - RNA, 20 nt, synthetic construct
  source 1..20: mol_type = other RNA
aggtaccagagacagagacg

SEQ ID NO: 16495 - RNA, 20 nt, synthetic construct
  source 1..20: mol_type = other RNA
ggtaccagagacagagacgt

SEQ ID NO: 16496 - RNA, 20 nt, synthetic construct
  source 1..20: mol_type = other RNA
gtaccagagacagagacgtg

SEQ ID NO: 16497 - RNA, 20 nt, synthetic construct
  source 1..20: mol_type = other RNA
gggccccacgtctctgtctc

SEQ ID NO: 16498 - RNA, 20 nt, synthetic construct
  source 1..20: mol_type = other RNA
acagagacgtggggcccatg

SEQ ID NO: 16499 - RNA, 20 nt, synthetic construct
  source 1..20: mol_type = other RNA
gcccatgcggtgtaaaaaac

SEQ ID NO: 16500 - RNA, 20 nt, synthetic construct
  source 1..20: mol_type = other RNA
cccatgcggtgtaaaaaacc

SEQ ID NO: 16501 - RNA, 20 nt, synthetic construct
  source 1..20: mol_type = other RNA
atgcggtgtaaaaaaccggg

SEQ ID NO: 16502 - RNA, 20 nt, synthetic construct
  source 1..20: mol_type = other RNA
cccggttttttacaccgcat

SEQ ID NO: 16503 - RNA, 20 nt, synthetic construct
  source 1..20: mol_type = other RNA
tcccggttttttacaccgca

SEQ ID NO: 16504 - RNA, 20 nt, synthetic construct
  source 1..20: mol_type = other RNA
aaaaaccgggaggtaccttc

SEQ ID NO: 16505 - RNA, 20 nt, synthetic construct
  source 1..20: mol_type = other RNA
tgggtcctgaaggtacctcc

SEQ ID NO: 16506 - RNA, 20 nt, synthetic construct
  source 1..20: mol_type = other RNA
gtaccttcaggacccacagc

SEQ ID NO: 16507 - RNA, 20 nt, synthetic construct
  source 1..20: mol_type = other RNA
taccttcaggacccacagct

SEQ ID NO: 16508 - RNA, 20 nt, synthetic construct
  source 1..20: mol_type = other RNA
ggcccagctgtgggtcctga

SEQ ID NO: 16509 - RNA, 20 nt, synthetic construct
  source 1..20: mol_type = other RNA
ggacccacagctgggcctca

SEQ ID NO: 16510 - RNA, 20 nt, synthetic construct
  source 1..20: mol_type = other RNA
tggccctgaggcccagctgt

SEQ ID NO: 16511 - RNA, 20 nt, synthetic construct
  source 1..20: mol_type = other RNA
gtggccctgaggcccagctg

SEQ ID NO: 16512 - RNA, 20 nt, synthetic construct
  source 1..20: mol_type = other RNA
ctgggcctcagggccacagc

SEQ ID NO: 16513 - RNA, 20 nt, synthetic construct
  source 1..20: mol_type = other RNA
tgggcctcagggccacagct

SEQ ID NO: 16514 - RNA, 20 nt, synthetic construct
  source 1..20: mol_type = other RNA
gggcctcagggccacagctg

SEQ ID NO: 16515 - RNA, 20 nt, synthetic construct
  source 1..20: mol_type = other RNA
tcagggccacagctggggtt

SEQ ID NO: 16516 - RNA, 20 nt, synthetic construct
  source 1..20: mol_type = other RNA
aaaccccagctgtggccctg

SEQ ID NO: 16517 - RNA, 20 nt, synthetic construct
  source 1..20: mol_type = other RNA
tgttcaccaaaccccagctg

SEQ ID NO: 16518 - RNA, 20 nt, synthetic construct
  source 1..20: mol_type = other RNA
gcactgaagtatgaagtgca

SEQ ID NO: 16519 - RNA, 20 nt, synthetic construct
  source 1..20: mol_type = other RNA
acttcagtgcccgccagttc

SEQ ID NO: 16520 - RNA, 20 nt, synthetic construct
  source 1..20: mol_type = other RNA
gcccgccagttcaggacatt

SEQ ID NO: 16521 - RNA, 20 nt, synthetic construct
  source 1..20: mol_type = other RNA
tcctaatgtcctgaactggc

SEQ ID NO: 16522 - RNA, 20 nt, synthetic construct
  source 1..20: mol_type = other RNA
gtcctaatgtcctgaactgg

SEQ ID NO: 16523 - RNA, 20 nt, synthetic construct
  source 1..20: mol_type = other RNA
gttcaggacattaggactga

SEQ ID NO: 16524 - RNA, 20 nt, synthetic construct
  source 1..20: mol_type = other RNA
ttcaggacattaggactgaa

SEQ ID NO: 16525 - RNA, 20 nt, synthetic construct
  source 1..20: mol_type = other RNA
tcagtcctaatgtcctgaac

SEQ ID NO: 16526 - RNA, 20 nt, synthetic construct
  source 1..20: mol_type = other RNA
gaagggcccgccaagataga

SEQ ID NO: 16527 - RNA, 20 nt, synthetic construct
  source 1..20: mol_type = other RNA
ttaacaccatctatcttggc

SEQ ID NO: 16528 - RNA, 20 nt, synthetic construct
  source 1..20: mol_type = other RNA
attaacaccatctatcttgg

SEQ ID NO: 16529 - RNA, 20 nt, synthetic construct
  source 1..20: mol_type = other RNA
gagattaacaccatctatct

SEQ ID NO: 16530 - RNA, 20 nt, synthetic construct
  source 1..20: mol_type = other RNA
tagatggtgttaatctcatc

SEQ ID NO: 16531 - RNA, 20 nt, synthetic construct
  source 1..20: mol_type = other RNA
cattggaaatgtgaacatgt

SEQ ID NO: 16532 - RNA, 20 nt, synthetic construct
  source 1..20: mol_type = other RNA
acattggaaatgtgaacatg

SEQ ID NO: 16533 - RNA, 20 nt, synthetic construct
  source 1..20: mol_type = other RNA
catttccaatgtctcccacc

SEQ ID NO: 16534 - RNA, 20 nt, synthetic construct
  source 1..20: mol_type = other RNA
atttccaatgtctcccacca

SEQ ID NO: 16535 - RNA, 20 nt, synthetic construct
  source 1..20: mol_type = other RNA
caatgtctcccaccagggac

SEQ ID NO: 16536 - RNA, 20 nt, synthetic construct
  source 1..20: mol_type = other RNA
cagtccctggtgggagacat

SEQ ID NO: 16537 - RNA, 20 nt, synthetic construct
  source 1..20: mol_type = other RNA
gaaggaagccagtccctggt

SEQ ID NO: 16538 - RNA, 20 nt, synthetic construct
  source 1..20: mol_type = other RNA
tgaaggaagccagtccctgg

SEQ ID NO: 16539 - RNA, 20 nt, synthetic construct
  source 1..20: mol_type = other RNA
ctttgaaggaagccagtccc

SEQ ID NO: 16540 - RNA, 20 nt, synthetic construct
  source 1..20: mol_type = other RNA
tccttcaaagttcccaccga

SEQ ID NO: 16541 - RNA, 20 nt, synthetic construct
  source 1..20: mol_type = other RNA
tccttcggtgggaactttga

SEQ ID NO: 16542 - RNA, 20 nt, synthetic construct
  source 1..20: mol_type = other RNA
aggagcaggattccttcggt

SEQ ID NO: 16543 - RNA, 20 nt, synthetic construct
  source 1..20: mol_type = other RNA
caggagcaggattccttcgg

SEQ ID NO: 16544 - RNA, 20 nt, synthetic construct
  source 1..20: mol_type = other RNA
gggcaggagcaggattcctt

SEQ ID NO: 16545 - RNA, 20 nt, synthetic construct
  source 1..20: mol_type = other RNA
catcatcttggggcaggagc

SEQ ID NO: 16546 - RNA, 20 nt, synthetic construct
  source 1..20: mol_type = other RNA
agcaagcatcatcttggggc

SEQ ID NO: 16547 - RNA, 20 nt, synthetic construct
  source 1..20: mol_type = other RNA
cagaagcaagcatcatcttg

SEQ ID NO: 16548 - RNA, 20 nt, synthetic construct
  source 1..20: mol_type = other RNA
gcagaagcaagcatcatctt

SEQ ID NO: 16549 - RNA, 20 nt, synthetic construct
  source 1..20: mol_type = other RNA
ggcagaagcaagcatcatct

SEQ ID NO: 16550 - RNA, 20 nt, synthetic construct
  source 1..20: mol_type = other RNA
gaagaagggatacactgtgg

SEQ ID NO: 16551 - RNA, 20 nt, synthetic construct
  source 1..20: mol_type = other RNA
tgaagaagggatacactgtg

SEQ ID NO: 16552 - RNA, 20 nt, synthetic construct
  source 1..20: mol_type = other RNA
ctgaagaagggatacactgt

SEQ ID NO: 16553 - RNA, 20 nt, synthetic construct
  source 1..20: mol_type = other RNA
tctgaagaagggatacactg

SEQ ID NO: 16554 - RNA, 20 nt, synthetic construct
  source 1..20: mol_type = other RNA
cttcagactcttcctcaccc

SEQ ID NO: 16555 - RNA, 20 nt, synthetic construct
  source 1..20: mol_type = other RNA
ttcagactcttcctcaccct

SEQ ID NO: 16556 - RNA, 20 nt, synthetic construct
  source 1..20: mol_type = other RNA
tagatgggaagcccagggtg

SEQ ID NO: 16557 - RNA, 20 nt, synthetic construct
  source 1..20: mol_type = other RNA
ctgggtagatgggaagccca

SEQ ID NO: 16558 - RNA, 20 nt, synthetic construct
  source 1..20: mol_type = other RNA
tctgggtagatgggaagccc

SEQ ID NO: 16559 - RNA, 20 nt, synthetic construct
  source 1..20: mol_type = other RNA
tcgtggagttctgggtagat

SEQ ID NO: 16560 - RNA, 20 nt, synthetic construct
  source 1..20: mol_type = other RNA
atcgtggagttctgggtaga

SEQ ID NO: 16561 - RNA, 20 nt, synthetic construct
  source 1..20: mol_type = other RNA
ccagaactccacgatccctg

SEQ ID NO: 16562 - RNA, 20 nt, synthetic construct
  source 1..20: mol_type = other RNA
gaactccacgatccctgagg

SEQ ID NO: 16563 - RNA, 20 nt, synthetic construct
  source 1..20: mol_type = other RNA
ctcagggatcgtggagttct

SEQ ID NO: 16564 - RNA, 20 nt, synthetic construct
  source 1..20: mol_type = other RNA
cctcagggatcgtggagttc

SEQ ID NO: 16565 - RNA, 20 nt, synthetic construct
  source 1..20: mol_type = other RNA
ggagtccgcctcagggatcg

SEQ ID NO: 16566 - RNA, 20 nt, synthetic construct
  source 1..20: mol_type = other RNA
caagctgggagtccgcctca

SEQ ID NO: 16567 - RNA, 20 nt, synthetic construct
  source 1..20: mol_type = other RNA
acaagctgggagtccgcctc

SEQ ID NO: 16568 - RNA, 20 nt, synthetic construct
  source 1..20: mol_type = other RNA
cagcttgtacaaatgtgtac

SEQ ID NO: 16569 - RNA, 20 nt, synthetic construct
  source 1..20: mol_type = other RNA
agtacacatttgtacaagct

SEQ ID NO: 16570 - RNA, 20 nt, synthetic construct
  source 1..20: mol_type = other RNA
cagtacacatttgtacaagc

SEQ ID NO: 16571 - RNA, 20 nt, synthetic construct
  source 1..20: mol_type = other RNA
actggagctactgtgacttc

SEQ ID NO: 16572 - RNA, 20 nt, synthetic construct
  source 1..20: mol_type = other RNA
tgggtctgaaatattattcg

SEQ ID NO: 16573 - RNA, 20 nt, synthetic construct
  source 1..20: mol_type = other RNA
gatacagttttacagtgggt

SEQ ID NO: 16574 - RNA, 20 nt, synthetic construct
  source 1..20: mol_type = other RNA
ggatacagttttacagtggg

SEQ ID NO: 16575 - RNA, 20 nt, synthetic construct
  source 1..20: mol_type = other RNA
ataggatacagttttacagt

SEQ ID NO: 16576 - RNA, 20 nt, synthetic construct
  source 1..20: mol_type = other RNA
tataggatacagttttacag

SEQ ID NO: 16577 - RNA, 20 nt, synthetic construct
  source 1..20: mol_type = other RNA
atattttggtctaaggatat

SEQ ID NO: 16578 - RNA, 20 nt, synthetic construct
  source 1..20: mol_type = other RNA
gattctcatattttggtcta

SEQ ID NO: 16579 - RNA, 20 nt, synthetic construct
  source 1..20: mol_type = other RNA
acaatgagattctcatattt

SEQ ID NO: 16580 - RNA, 20 nt, synthetic construct
  source 1..20: mol_type = other RNA
aatctcattgtcttgtctct

SEQ ID NO: 16581 - RNA, 20 nt, synthetic construct
  source 1..20: mol_type = other RNA
ctcattgtcttgtctcttgg

SEQ ID NO: 16582 - RNA, 20 nt, synthetic construct
  source 1..20: mol_type = other RNA
acgagaaaatactgtaccca

SEQ ID NO: 16583 - RNA, 20 nt, synthetic construct
  source 1..20: mol_type = other RNA
cgagaaaatactgtacccac

SEQ ID NO: 16584 - RNA, 20 nt, synthetic construct
  source 1..20: mol_type = other RNA
aatactgtacccacgggtcg

SEQ ID NO: 16585 - RNA, 20 nt, synthetic construct
  source 1..20: mol_type = other RNA
cggaactgtcctcgacccgt

SEQ ID NO: 16586 - RNA, 20 nt, synthetic construct
  source 1..20: mol_type = other RNA
acggaactgtcctcgacccg

SEQ ID NO: 16587 - RNA, 20 nt, synthetic construct
  source 1..20: mol_type = other RNA
aggacagttccgtgtagaag

SEQ ID NO: 16588 - RNA, 20 nt, synthetic construct
  source 1..20: mol_type = other RNA
acagttccgtgtagaagtgg

SEQ ID NO: 16589 - RNA, 20 nt, synthetic construct
  source 1..20: mol_type = other RNA
tgtgtgcctccacttctaca

SEQ ID NO: 16590 - RNA, 20 nt, synthetic construct
  source 1..20: mol_type = other RNA
gaagtggaggcacacagtga

SEQ ID NO: 16591 - RNA, 20 nt, synthetic construct
  source 1..20: mol_type = other RNA
cacacagtgaaggctttgag

SEQ ID NO: 16592 - RNA, 20 nt, synthetic construct
  source 1..20: mol_type = other RNA
gctttgagaggcttcgttaa

SEQ ID NO: 16593 - RNA, 20 nt, synthetic construct
  source 1..20: mol_type = other RNA
gcttcgttaacggtgctttg

SEQ ID NO: 16594 - RNA, 20 nt, synthetic construct
  source 1..20: mol_type = other RNA
cttcgttaacggtgctttga

SEQ ID NO: 16595 - RNA, 20 nt, synthetic construct
  source 1..20: mol_type = other RNA
cggtgctttgagggatacat

SEQ ID NO: 16596 - RNA, 20 nt, synthetic construct
  source 1..20: mol_type = other RNA
ataggaagtatccgactctt

SEQ ID NO: 16597 - RNA, 20 nt, synthetic construct
  source 1..20: mol_type = other RNA
taggaagtatccgactcttt

SEQ ID NO: 16598 - RNA, 20 nt, synthetic construct
  source 1..20: mol_type = other RNA
ttttgtgtttcccaaagagt

SEQ ID NO: 16599 - RNA, 20 nt, synthetic construct
  source 1..20: mol_type = other RNA
gctcacagacatgtcgagga

SEQ ID NO: 16600 - RNA, 20 nt, synthetic construct
  source 1..20: mol_type = other RNA
tctggctcacagacatgtcg

SEQ ID NO: 16601 - RNA, 20 nt, synthetic construct
  source 1..20: mol_type = other RNA
gaaaaacaagcaaatgtgag

SEQ ID NO: 16602 - RNA, 20 nt, synthetic construct
  source 1..20: mol_type = other RNA
ctcacatttgcttgtttttc

SEQ ID NO: 16603 - RNA, 20 nt, synthetic construct
  source 1..20: mol_type = other RNA
aaattctatacgtaagtgag

SEQ ID NO: 16604 - RNA, 20 nt, synthetic construct
  source 1..20: mol_type = other RNA
taaattctatacgtaagtga

SEQ ID NO: 16605 - RNA, 20 nt, synthetic construct
  source 1..20: mol_type = other RNA
ttaaattctatacgtaagtg

SEQ ID NO: 16606 - RNA, 20 nt, synthetic construct
  source 1..20: mol_type = other RNA
gtggtgtgtaactggagaag

SEQ ID NO: 16607 - RNA, 20 nt, synthetic construct
  source 1..20: mol_type = other RNA
agactgtatgaacagaacag

SEQ ID NO: 16608 - RNA, 20 nt, synthetic construct
  source 1..20: mol_type = other RNA
tgatctgaggtatgggggtg

SEQ ID NO: 16609 - RNA, 20 nt, synthetic construct
  source 1..20: mol_type = other RNA
ttgatctgaggtatgggggt

SEQ ID NO: 16610 - RNA, 20 nt, synthetic construct
  source 1..20: mol_type = other RNA
tttgatctgaggtatggggg

SEQ ID NO: 16611 - RNA, 20 nt, synthetic construct
  source 1..20: mol_type = other RNA
agatttgatctgaggtatgg

SEQ ID NO: 16612 - RNA, 20 nt, synthetic construct
  source 1..20: mol_type = other RNA
gagatttgatctgaggtatg

SEQ ID NO: 16613 - RNA, 20 nt, synthetic construct
  source 1..20: mol_type = other RNA
agagatttgatctgaggtat

SEQ ID NO: 16614 - RNA, 20 nt, synthetic construct
  source 1..20: mol_type = other RNA
gagagatttgatctgaggta

SEQ ID NO: 16615 - RNA, 20 nt, synthetic construct
  source 1..20: mol_type = other RNA
tatgggagagatttgatctg

SEQ ID NO: 16616 - RNA, 20 nt, synthetic construct
  source 1..20: mol_type = other RNA
atcaaatctctcccatagcc

SEQ ID NO: 16617 - RNA, 20 nt, synthetic construct
  source 1..20: mol_type = other RNA
tcaaatctctcccatagcct

SEQ ID NO: 16618 - RNA, 20 nt, synthetic construct
  source 1..20: mol_type = other RNA
caaatctctcccatagcctg

SEQ ID NO: 16619 - RNA, 20 nt, synthetic construct
  source 1..20: mol_type = other RNA
atctctcccatagcctgggg

SEQ ID NO: 16620 - RNA, 20 nt, synthetic construct
  source 1..20: mol_type = other RNA
taagggccaccccaggctat

SEQ ID NO: 16621 - RNA, 20 nt, synthetic construct
  source 1..20: mol_type = other RNA
gtaagggccaccccaggcta

SEQ ID NO: 16622 - RNA, 20 nt, synthetic construct
  source 1..20: mol_type = other RNA
tggggtggcccttacctgtc

SEQ ID NO: 16623 - RNA, 20 nt, synthetic construct
  source 1..20: mol_type = other RNA
agacaggtaagggccacccc

SEQ ID NO: 16624 - RNA, 20 nt, synthetic construct
  source 1..20: mol_type = other RNA
gcttttggccagacaggtaa

SEQ ID NO: 16625 - RNA, 20 nt, synthetic construct
  source 1..20: mol_type = other RNA
tgcttttggccagacaggta

SEQ ID NO: 16626 - RNA, 20 nt, synthetic construct
  source 1..20: mol_type = other RNA
tctggccaaaagcatgagag

SEQ ID NO: 16627 - RNA, 20 nt, synthetic construct
  source 1..20: mol_type = other RNA
tctcatgcttttggccagac

SEQ ID NO: 16628 - RNA, 20 nt, synthetic construct
  source 1..20: mol_type = other RNA
gccaaaagcatgagagaggc

SEQ ID NO: 16629 - RNA, 20 nt, synthetic construct
  source 1..20: mol_type = other RNA
accagcctctctcatgcttt

SEQ ID NO: 16630 - RNA, 20 nt, synthetic construct
  source 1..20: mol_type = other RNA
gaaacacaacagcttctcca

SEQ ID NO: 16631 - RNA, 20 nt, synthetic construct
  source 1..20: mol_type = other RNA
ggagaagctgttgtgtttct

SEQ ID NO: 16632 - RNA, 20 nt, synthetic construct
  source 1..20: mol_type = other RNA
ctggcagcaggacgtgacca

SEQ ID NO: 16633 - RNA, 20 nt, synthetic construct
  source 1..20: mol_type = other RNA
gtcctgctgccagtgataca

SEQ ID NO: 16634 - RNA, 20 nt, synthetic construct
  source 1..20: mol_type = other RNA
tcctgctgccagtgatacaa

SEQ ID NO: 16635 - RNA, 20 nt, synthetic construct
  source 1..20: mol_type = other RNA
gcccttgtatcactggcagc

SEQ ID NO: 16636 - RNA, 20 nt, synthetic construct
  source 1..20: mol_type = other RNA
aattcaggcccttgtatcac

SEQ ID NO: 16637 - RNA, 20 nt, synthetic construct
  source 1..20: mol_type = other RNA
agggcctgaattcactcctt

SEQ ID NO: 16638 - RNA, 20 nt, synthetic construct
  source 1..20: mol_type = other RNA
ttttccaaaggagtgaattc

SEQ ID NO: 16639 - RNA, 20 nt, synthetic construct
  source 1..20: mol_type = other RNA
tcctttggaaaagatgtatt

SEQ ID NO: 16640 - RNA, 20 nt, synthetic construct
  source 1..20: mol_type = other RNA
gccgaatacatcttttccaa

SEQ ID NO: 16641 - RNA, 20 nt, synthetic construct
  source 1..20: mol_type = other RNA
atgtattcggctgaaagttc

SEQ ID NO: 16642 - RNA, 20 nt, synthetic construct
  source 1..20: mol_type = other RNA
tgtattcggctgaaagttca

SEQ ID NO: 16643 - RNA, 20 nt, synthetic construct
  source 1..20: mol_type = other RNA
gtattcggctgaaagttcag

SEQ ID NO: 16644 - RNA, 20 nt, synthetic construct
  source 1..20: mol_type = other RNA
agctctaaggcaagagatct

SEQ ID NO: 16645 - RNA, 20 nt, synthetic construct
  source 1..20: mol_type = other RNA
tagagctacctcctcctgcc

SEQ ID NO: 16646 - RNA, 20 nt, synthetic construct
  source 1..20: mol_type = other RNA
ggcaggaggaggtagctcta

SEQ ID NO: 16647 - RNA, 20 nt, synthetic construct
  source 1..20: mol_type = other RNA
atataaatccaggcaggagg

SEQ ID NO: 16648 - RNA, 20 nt, synthetic construct
  source 1..20: mol_type = other RNA
tggatataaatccaggcagg

SEQ ID NO: 16649 - RNA, 20 nt, synthetic construct
  source 1..20: mol_type = other RNA
ctttggatataaatccaggc

SEQ ID NO: 16650 - RNA, 20 nt, synthetic construct
  source 1..20: mol_type = other RNA
gatttatatccaaagcagta

SEQ ID NO: 16651 - RNA, 20 nt, synthetic construct
  source 1..20: mol_type = other RNA
actgctttggatataaatcc

SEQ ID NO: 16652 - RNA, 20 nt, synthetic construct
  source 1..20: mol_type = other RNA
cgcaaactcccttactgctt

SEQ ID NO: 16653 - RNA, 20 nt, synthetic construct
  source 1..20: mol_type = other RNA
ttggaaaattatttacatag

SEQ ID NO: 16654 - RNA, 20 nt, synthetic construct
  source 1..20: mol_type = other RNA
aattttccaacattgcttgt

SEQ ID NO: 16655 - RNA, 20 nt, synthetic construct
  source 1..20: mol_type = other RNA
attttccaacattgcttgtt

SEQ ID NO: 16656 - RNA, 20 nt, synthetic construct
  source 1..20: mol_type = other RNA
ttttccaacattgcttgttg

SEQ ID NO: 16657 - RNA, 20 nt, synthetic construct
  source 1..20: mol_type = other RNA
ccaacattgcttgttggggc

SEQ ID NO: 16658 - RNA, 20 nt, synthetic construct
  source 1..20: mol_type = other RNA
cctgccccaacaagcaatgt

SEQ ID NO: 16659 - RNA, 20 nt, synthetic construct
  source 1..20: mol_type = other RNA
tggggcaggtgtcagagctt

SEQ ID NO: 16660 - RNA, 20 nt, synthetic construct
  source 1..20: mol_type = other RNA
ggggcaggtgtcagagcttc

SEQ ID NO: 16661 - RNA, 20 nt, synthetic construct
  source 1..20: mol_type = other RNA
ggtgtcagagcttcgggaag

SEQ ID NO: 16662 - RNA, 20 nt, synthetic construct
  source 1..20: mol_type = other RNA
gtgtcagagcttcgggaaga

SEQ ID NO: 16663 - RNA, 20 nt, synthetic construct
  source 1..20: mol_type = other RNA
tgtcagagcttcgggaagag

SEQ ID NO: 16664 - RNA, 20 nt, synthetic construct
  source 1..20: mol_type = other RNA
attggtaattcagtagtcat

SEQ ID NO: 16665 - RNA, 20 nt, synthetic construct
  source 1..20: mol_type = other RNA
aattaccaattctttatgac

SEQ ID NO: 16666 - RNA, 20 nt, synthetic construct
  source 1..20: mol_type = other RNA
tttttcctgtcataaagaat

SEQ ID NO: 16667 - RNA, 20 nt, synthetic construct
  source 1..20: mol_type = other RNA
gaaaaatgaagaaatctctc

SEQ ID NO: 16668 - RNA, 20 nt, synthetic construct
  source 1..20: mol_type = other RNA
aaaaatgaagaaatctctca

SEQ ID NO: 16669 - RNA, 20 nt, synthetic construct
  source 1..20: mol_type = other RNA
aatctctcagggctccactt

SEQ ID NO: 16670 - RNA, 20 nt, synthetic construct
  source 1..20: mol_type = other RNA
cgcaggatagatagccaaag

SEQ ID NO: 16671 - RNA, 20 nt, synthetic construct
  source 1..20: mol_type = other RNA
tatctatcctgcgaaaataa

SEQ ID NO: 16672 - RNA, 20 nt, synthetic construct
  source 1..20: mol_type = other RNA
atctatcctgcgaaaataat

SEQ ID NO: 16673 - RNA, 20 nt, synthetic construct
  source 1..20: mol_type = other RNA
cctgcgaaaataatgggaaa

SEQ ID NO: 16674 - RNA, 20 nt, synthetic construct
  source 1..20: mol_type = other RNA
ccatttcccattattttcgc

SEQ ID NO: 16675 - RNA, 20 nt, synthetic construct
  source 1..20: mol_type = other RNA
atggtaacatattaaacgag

SEQ ID NO: 16676 - RNA, 20 nt, synthetic construct
  source 1..20: mol_type = other RNA
atattaaacgagtggccatc

SEQ ID NO: 16677 - RNA, 20 nt, synthetic construct
  source 1..20: mol_type = other RNA
tattaaacgagtggccatct

SEQ ID NO: 16678 - RNA, 20 nt, synthetic construct
  source 1..20: mol_type = other RNA
agtggccatctgggtgcacg

SEQ ID NO: 16679 - RNA, 20 nt, synthetic construct
  source 1..20: mol_type = other RNA
agctaccacgtgcacccaga

SEQ ID NO: 16680 - RNA, 20 nt, synthetic construct
  source 1..20: mol_type = other RNA
ggctgaagtaggtgttggag

SEQ ID NO: 16681 - RNA, 20 nt, synthetic construct
  source 1..20: mol_type = other RNA
atttgggctgaagtaggtgt

SEQ ID NO: 16682 - RNA, 20 nt, synthetic construct
  source 1..20: mol_type = other RNA
tctatgatttgggctgaagt

SEQ ID NO: 16683 - RNA, 20 nt, synthetic construct
  source 1..20: mol_type = other RNA
caaatcatagagtttgacaa

SEQ ID NO: 16684 - RNA, 20 nt, synthetic construct
  source 1..20: mol_type = other RNA
tttgtcaaactctatgattt

SEQ ID NO: 16685 - RNA, 20 nt, synthetic construct
  source 1..20: mol_type = other RNA
ctttgtcaaactctatgatt

SEQ ID NO: 16686 - RNA, 20 nt, synthetic construct
  source 1..20: mol_type = other RNA
aaaggaaatctgacagcttc

SEQ ID NO: 16687 - RNA, 20 nt, synthetic construct
  source 1..20: mol_type = other RNA
aatctgacagcttctggaga

SEQ ID NO: 16688 - RNA, 20 nt, synthetic construct
  source 1..20: mol_type = other RNA
gtaaataagcaaattgaaag

SEQ ID NO: 16689 - RNA, 20 nt, synthetic construct
  source 1..20: mol_type = other RNA
tgtaaataagcaaattgaaa

SEQ ID NO: 16690 - RNA, 20 nt, synthetic construct
  source 1..20: mol_type = other RNA
caatttgcttatttacagac

SEQ ID NO: 16691 - RNA, 20 nt, synthetic construct
  source 1..20: mol_type = other RNA
aatttgcttatttacagact

SEQ ID NO: 16692 - RNA, 20 nt, synthetic construct
  source 1..20: mol_type = other RNA
tatttacagactgggaaatg

SEQ ID NO: 16693 - RNA, 20 nt, synthetic construct
  source 1..20: mol_type = other RNA
acatgctcctcccagagcca

SEQ ID NO: 16694 - RNA, 20 nt, synthetic construct
  source 1..20: mol_type = other RNA
aatgtgtccatggctctggg

SEQ ID NO: 16695 - RNA, 20 nt, synthetic construct
  source 1..20: mol_type = other RNA
aaaaatgtgtccatggctct

SEQ ID NO: 16696 - RNA, 20 nt, synthetic construct
  source 1..20: mol_type = other RNA
aaaaaatgtgtccatggctc

SEQ ID NO: 16697 - RNA, 20 nt, synthetic construct
  source 1..20: mol_type = other RNA
ataataaaaaaatgtgtcca

SEQ ID NO: 16698 - RNA, 20 nt, synthetic construct
  source 1..20: mol_type = other RNA
attattatactttaagtttt

SEQ ID NO: 16699 - RNA, 20 nt, synthetic construct
  source 1..20: mol_type = other RNA
ttattatactttaagtttta

SEQ ID NO: 16700 - RNA, 20 nt, synthetic construct
  source 1..20: mol_type = other RNA
ggtacatgtgcacaatgtgc

SEQ ID NO: 16701 - RNA, 20 nt, synthetic construct
  source 1..20: mol_type = other RNA
tatgtatacatgtgccatgc

SEQ ID NO: 16702 - RNA, 20 nt, synthetic construct
  source 1..20: mol_type = other RNA
atgggtgcagcacaccagca

SEQ ID NO: 16703 - RNA, 20 nt, synthetic construct
  source 1..20: mol_type = other RNA
ttaactcatcatttagcatt

SEQ ID NO: 16704 - RNA, 20 nt, synthetic construct
  source 1..20: mol_type = other RNA
atgctaaatgatgagttaat

SEQ ID NO: 16705 - RNA, 20 nt, synthetic construct
  source 1..20: mol_type = other RNA
aatgctaaatgatgagttaa

SEQ ID NO: 16706 - RNA, 20 nt, synthetic construct
  source 1..20: mol_type = other RNA
tggggtggggggagggggga

SEQ ID NO: 16707 - RNA, 20 nt, synthetic construct
  source 1..20: mol_type = other RNA
gtggggtggggggagggggg

SEQ ID NO: 16708 - RNA, 20 nt, synthetic construct
  source 1..20: mol_type = other RNA
gttgtggggtggggggaggg

SEQ ID NO: 16709 - RNA, 20 nt, synthetic construct
  source 1..20: mol_type = other RNA
tgttgtggggtggggggagg

SEQ ID NO: 16710 - RNA, 20 nt, synthetic construct
  source 1..20: mol_type = other RNA
ctgttgtggggtggggggag

SEQ ID NO: 16711 - RNA, 20 nt, synthetic construct
  source 1..20: mol_type = other RNA
actgttgtggggtgggggga

SEQ ID NO: 16712 - RNA, 20 nt, synthetic construct
  source 1..20: mol_type = other RNA
gactgttgtggggtgggggg

SEQ ID NO: 16713 - RNA, 20 nt, synthetic construct
  source 1..20: mol_type = other RNA
ggggactgttgtggggtggg

SEQ ID NO: 16714 - RNA, 20 nt, synthetic construct
  source 1..20: mol_type = other RNA
tggggactgttgtggggtgg

SEQ ID NO: 16715 - RNA, 20 nt, synthetic construct
  source 1..20: mol_type = other RNA
ctggggactgttgtggggtg

SEQ ID NO: 16716 - RNA, 20 nt, synthetic construct
  source 1..20: mol_type = other RNA
tctggggactgttgtggggt

SEQ ID NO: 16717 - RNA, 20 nt, synthetic construct
  source 1..20: mol_type = other RNA
ctctggggactgttgtgggg

SEQ ID NO: 16718 - RNA, 20 nt, synthetic construct
  source 1..20: mol_type = other RNA
acactctggggactgttgtg

SEQ ID NO: 16719 - RNA, 20 nt, synthetic construct
  source 1..20: mol_type = other RNA
cacactctggggactgttgt

SEQ ID NO: 16720 - RNA, 20 nt, synthetic construct
  source 1..20: mol_type = other RNA
tcacactctggggactgttg

SEQ ID NO: 16721 - RNA, 20 nt, synthetic construct
  source 1..20: mol_type = other RNA
aaggggaacatcacactctg

SEQ ID NO: 16722 - RNA, 20 nt, synthetic construct
  source 1..20: mol_type = other RNA
gaaggggaacatcacactct

SEQ ID NO: 16723 - RNA, 20 nt, synthetic construct
  source 1..20: mol_type = other RNA
ggaaggggaacatcacactc

SEQ ID NO: 16724 - RNA, 20 nt, synthetic construct
  source 1..20: mol_type = other RNA
gaatacttggacacaggaag

SEQ ID NO: 16725 - RNA, 20 nt, synthetic construct
  source 1..20: mol_type = other RNA
agaatacttggacacaggaa

SEQ ID NO: 16726 - RNA, 20 nt, synthetic construct
  source 1..20: mol_type = other RNA
gagaatacttggacacagga

SEQ ID NO: 16727 - RNA, 20 nt, synthetic construct
  source 1..20: mol_type = other RNA
caatgagaatacttggacac

SEQ ID NO: 16728 - RNA, 20 nt, synthetic construct
  source 1..20: mol_type = other RNA
aattgaacaatgagaatact

SEQ ID NO: 16729 - RNA, 20 nt, synthetic construct
  source 1..20: mol_type = other RNA
catctatgagtgagaacacg

SEQ ID NO: 16730 - RNA, 20 nt, synthetic construct
  source 1..20: mol_type = other RNA
gcgtgttctcactcatagat

SEQ ID NO: 16731 - RNA, 20 nt, synthetic construct
  source 1..20: mol_type = other RNA
cgcgtgttctcactcataga

SEQ ID NO: 16732 - RNA, 20 nt, synthetic construct
  source 1..20: mol_type = other RNA
gagtgagaacacgcggtgtt

SEQ ID NO: 16733 - RNA, 20 nt, synthetic construct
  source 1..20: mol_type = other RNA
gcggtgtttggttttttgca

SEQ ID NO: 16734 - RNA, 20 nt, synthetic construct
  source 1..20: mol_type = other RNA
tcttaataagtgtactcaat

SEQ ID NO: 16735 - RNA, 20 nt, synthetic construct
  source 1..20: mol_type = other RNA
taagaactctctagacatct

SEQ ID NO: 16736 - RNA, 20 nt, synthetic construct
  source 1..20: mol_type = other RNA
gacatcttggcactaaatga

SEQ ID NO: 16737 - RNA, 20 nt, synthetic construct
  source 1..20: mol_type = other RNA
ttactggacttttactgtca

SEQ ID NO: 16738 - RNA, 20 nt, synthetic construct
  source 1..20: mol_type = other RNA
tttactggacttttactgtc

SEQ ID NO: 16739 - RNA, 20 nt, synthetic construct
  source 1..20: mol_type = other RNA
tgatcaggcacacattttac

SEQ ID NO: 16740 - RNA, 20 nt, synthetic construct
  source 1..20: mol_type = other RNA
ataatgctatgtctgtgatc

SEQ ID NO: 16741 - RNA, 20 nt, synthetic construct
  source 1..20: mol_type = other RNA
acatattcagagaaaaatgt

SEQ ID NO: 16742 - RNA, 20 nt, synthetic construct
  source 1..20: mol_type = other RNA
ctctgaatatgtaaagcttc

SEQ ID NO: 16743 - RNA, 20 nt, synthetic construct
  source 1..20: mol_type = other RNA
gaatatgtaaagcttcaggc

SEQ ID NO: 16744 - RNA, 20 nt, synthetic construct
  source 1..20: mol_type = other RNA
taaagcttcaggcaggagtc

SEQ ID NO: 16745 - RNA, 20 nt, synthetic construct
  source 1..20: mol_type = other RNA
tacttgaatcttgtgaatag

SEQ ID NO: 16746 - RNA, 20 nt, synthetic construct
  source 1..20: mol_type = other RNA
agattgacagacagtgtgga

SEQ ID NO: 16747 - RNA, 20 nt, synthetic construct
  source 1..20: mol_type = other RNA
aagattgacagacagtgtgg

SEQ ID NO: 16748 - RNA, 20 nt, synthetic construct
  source 1..20: mol_type = other RNA
agtaagattgacagacagtg

SEQ ID NO: 16749 - RNA, 20 nt, synthetic construct
  source 1..20: mol_type = other RNA
tttgaagagtgagttaagta

SEQ ID NO: 16750 - RNA, 20 nt, synthetic construct
  source 1..20: mol_type = other RNA
ttttgaagagtgagttaagt

SEQ ID NO: 16751 - RNA, 20 nt, synthetic construct
  source 1..20: mol_type = other RNA
ggacttgaggagcaaggaga

SEQ ID NO: 16752 - RNA, 20 nt, synthetic construct
  source 1..20: mol_type = other RNA
ttttggggacttgaggagca

SEQ ID NO: 16753 - RNA, 20 nt, synthetic construct
  source 1..20: mol_type = other RNA
aatgagattttggggacttg

SEQ ID NO: 16754 - RNA, 20 nt, synthetic construct
  source 1..20: mol_type = other RNA
aaagaataaatgagattttg

SEQ ID NO: 16755 - RNA, 20 nt, synthetic construct
  source 1..20: mol_type = other RNA
gaaagaataaatgagatttt

SEQ ID NO: 16756 - RNA, 20 nt, synthetic construct
  source 1..20: mol_type = other RNA
tgaaagaataaatgagattt

SEQ ID NO: 16757 - RNA, 20 nt, synthetic construct
  source 1..20: mol_type = other RNA
gcttctaacttctcaatgaa

SEQ ID NO: 16758 - RNA, 20 nt, synthetic construct
  source 1..20: mol_type = other RNA
ctctactacaaaggatacgg

SEQ ID NO: 16759 - RNA, 20 nt, synthetic construct
  source 1..20: mol_type = other RNA
agactctactacaaaggata

SEQ ID NO: 16760 - RNA, 20 nt, synthetic construct
  source 1..20: mol_type = other RNA
gctagaagactctactacaa

SEQ ID NO: 16761 - RNA, 20 nt, synthetic construct
  source 1..20: mol_type = other RNA
agagaatggatgttagggaa

SEQ ID NO: 16762 - RNA, 20 nt, synthetic construct
  source 1..20: mol_type = other RNA
gaagtagagaatggatgtta

SEQ ID NO: 16763 - RNA, 20 nt, synthetic construct
  source 1..20: mol_type = other RNA
agaagtagagaatggatgtt

SEQ ID NO: 16764 - RNA, 20 nt, synthetic construct
  source 1..20: mol_type = other RNA
ctcttatgagaagtagagaa

SEQ ID NO: 16765 - RNA, 20 nt, synthetic construct
  source 1..20: mol_type = other RNA
agaagaataacattttcagt

SEQ ID NO: 16766 - RNA, 20 nt, synthetic construct
  source 1..20: mol_type = other RNA
gaagaataacattttcagtt

SEQ ID NO: 16767 - RNA, 20 nt, synthetic construct
  source 1..20: mol_type = other RNA
aacattttcagttgggcgct

SEQ ID NO: 16768 - RNA, 20 nt, synthetic construct
  source 1..20: mol_type = other RNA
tgggaaatttggtgtttgag

SEQ ID NO: 16769 - RNA, 20 nt, synthetic construct
  source 1..20: mol_type = other RNA
ctgggaaatttggtgtttga

SEQ ID NO: 16770 - RNA, 20 nt, synthetic construct
  source 1..20: mol_type = other RNA
gctgggaaatttggtgtttg

SEQ ID NO: 16771 - RNA, 20 nt, synthetic construct
  source 1..20: mol_type = other RNA
acagtgggggctgggaaatt

SEQ ID NO: 16772 - RNA, 20 nt, synthetic construct
  source 1..20: mol_type = other RNA
tgcaagctacagtgggggct

SEQ ID NO: 16773 - RNA, 20 nt, synthetic construct
  source 1..20: mol_type = other RNA
ctgcaagctacagtgggggc

SEQ ID NO: 16774 - RNA, 20 nt, synthetic construct
  source 1..20: mol_type = other RNA
atcactgcaagctacagtgg

SEQ ID NO: 16775 - RNA, 20 nt, synthetic construct
  source 1..20: mol_type = other RNA
catcactgcaagctacagtg

SEQ ID NO: 16776 - RNA, 20 nt, synthetic construct
  source 1..20: mol_type = other RNA
tcatcactgcaagctacagt

SEQ ID NO: 16777 - RNA, 20 nt, synthetic construct
  source 1..20: mol_type = other RNA
atcatcactgcaagctacag

SEQ ID NO: 16778 - RNA, 20 nt, synthetic construct
  source 1..20: mol_type = other RNA
gtgatgatgtgattaaatta

SEQ ID NO: 16779 - RNA, 20 nt, synthetic construct
  source 1..20: mol_type = other RNA
caacgagatatgaacagaat

SEQ ID NO: 16780 - RNA, 20 nt, synthetic construct
  source 1..20: mol_type = other RNA
aacgagatatgaacagaata

SEQ ID NO: 16781 - RNA, 20 nt, synthetic construct
  source 1..20: mol_type = other RNA
ctattctgttcatatctcgt

SEQ ID NO: 16782 - RNA, 20 nt, synthetic construct
  source 1..20: mol_type = other RNA
acagaatagggaccatctct

SEQ ID NO: 16783 - RNA, 20 nt, synthetic construct
  source 1..20: mol_type = other RNA
taaagagcacaacctagaga

SEQ ID NO: 16784 - RNA, 20 nt, synthetic construct
  source 1..20: mol_type = other RNA
taggttgtgctctttaagaa

SEQ ID NO: 16785 - RNA, 20 nt, synthetic construct
  source 1..20: mol_type = other RNA
gaaaaagggggaagtgggag

SEQ ID NO: 16786 - RNA, 20 nt, synthetic construct
  source 1..20: mol_type = other RNA
ggaaaaagggggaagtggga

SEQ ID NO: 16787 - RNA, 20 nt, synthetic construct
  source 1..20: mol_type = other RNA
gggaaaaagggggaagtggg

SEQ ID NO: 16788 - RNA, 20 nt, synthetic construct
  source 1..20: mol_type = other RNA
aaagggaaaaagggggaagt

SEQ ID NO: 16789 - RNA, 20 nt, synthetic construct
  source 1..20: mol_type = other RNA
caaagggaaaaagggggaag

SEQ ID NO: 16790 - RNA, 20 nt, synthetic construct
  source 1..20: mol_type = other RNA
actagtcaaagggaaaaagg

SEQ ID NO: 16791 - RNA, 20 nt, synthetic construct
  source 1..20: mol_type = other RNA
tactagtcaaagggaaaaag

SEQ ID NO: 16792 - RNA, 20 nt, synthetic construct
  source 1..20: mol_type = other RNA
atactagtcaaagggaaaaa

SEQ ID NO: 16793 - RNA, 20 nt, synthetic construct
  source 1..20: mol_type = other RNA
aatactagtcaaagggaaaa

SEQ ID NO: 16794 - RNA, 20 nt, synthetic construct
  source 1..20: mol_type = other RNA
atgactgaatactagtcaaa

SEQ ID NO: 16795 - RNA, 20 nt, synthetic construct
  source 1..20: mol_type = other RNA
catgactgaatactagtcaa

SEQ ID NO: 16796 - RNA, 20 nt, synthetic construct
  source 1..20: mol_type = other RNA
tagtattcagtcatgatagc

SEQ ID NO: 16797 - RNA, 20 nt, synthetic construct
  source 1..20: mol_type = other RNA
tcagtcatgatagcaggaga

SEQ ID NO: 16798 - RNA, 20 nt, synthetic construct
  source 1..20: mol_type = other RNA
agatggaatagttcactttc

SEQ ID NO: 16799 - RNA, 20 nt, synthetic construct
  source 1..20: mol_type = other RNA
caagtgtaagctgcatgttg

SEQ ID NO: 16800 - RNA, 20 nt, synthetic construct
  source 1..20: mol_type = other RNA
aacatgcagcttacacttgc

SEQ ID NO: 16801 - RNA, 20 nt, synthetic construct
  source 1..20: mol_type = other RNA
tgtaagctgcatgttgaggt

SEQ ID NO: 16802 - RNA, 20 nt, synthetic construct
  source 1..20: mol_type = other RNA
gctgcatgttgaggttggca

SEQ ID NO: 16803 - RNA, 20 nt, synthetic construct
  source 1..20: mol_type = other RNA
tggcatggcaacaagataga

SEQ ID NO: 16804 - RNA, 20 nt, synthetic construct
  source 1..20: mol_type = other RNA
gcaacaagatagatggagcc

SEQ ID NO: 16805 - RNA, 20 nt, synthetic construct
  source 1..20: mol_type = other RNA
ggctccatacccaattatcc

SEQ ID NO: 16806 - RNA, 20 nt, synthetic construct
  source 1..20: mol_type = other RNA
tctccttcctccttatcgta

SEQ ID NO: 16807 - RNA, 20 nt, synthetic construct
  source 1..20: mol_type = other RNA
ctccttcctccttatcgtat

SEQ ID NO: 16808 - RNA, 20 nt, synthetic construct
  source 1..20: mol_type = other RNA
tcctccttatcgtatgggtt

SEQ ID NO: 16809 - RNA, 20 nt, synthetic construct
  source 1..20: mol_type = other RNA
aacccatacgataaggagga

SEQ ID NO: 16810 - RNA, 20 nt, synthetic construct
  source 1..20: mol_type = other RNA
gcctaacccatacgataagg

SEQ ID NO: 16811 - RNA, 20 nt, synthetic construct
  source 1..20: mol_type = other RNA
tttgcctaacccatacgata

SEQ ID NO: 16812 - RNA, 20 nt, synthetic construct
  source 1..20: mol_type = other RNA
gaaattttcttccagacagt

SEQ ID NO: 16813 - RNA, 20 nt, synthetic construct
  source 1..20: mol_type = other RNA
gaggtcacagtccaactgtc

SEQ ID NO: 16814 - RNA, 20 nt, synthetic construct
  source 1..20: mol_type = other RNA
ctgagtcctaccagctttgt

SEQ ID NO: 16815 - RNA, 20 nt, synthetic construct
  source 1..20: mol_type = other RNA
acaaagctggtaggactcag

SEQ ID NO: 16816 - RNA, 20 nt, synthetic construct
  source 1..20: mol_type = other RNA
gattctccaacaaagctggt

SEQ ID NO: 16817 - RNA, 20 nt, synthetic construct
  source 1..20: mol_type = other RNA
tctggattctccaacaaagc

SEQ ID NO: 16818 - RNA, 20 nt, synthetic construct
  source 1..20: mol_type = other RNA
aatccagatgtagatgagaa

SEQ ID NO: 16819 - RNA, 20 nt, synthetic construct
  source 1..20: mol_type = other RNA
acaccgttctcatctacatc

SEQ ID NO: 16820 - RNA, 20 nt, synthetic construct
  source 1..20: mol_type = other RNA
gatgagaacggtgttgccta

SEQ ID NO: 16821 - RNA, 20 nt, synthetic construct
  source 1..20: mol_type = other RNA
ctaaggccacacttcaagcc

SEQ ID NO: 16822 - RNA, 20 nt, synthetic construct
  source 1..20: mol_type = other RNA
ctggcttgaagtgtggcctt

SEQ ID NO: 16823 - RNA, 20 nt, synthetic construct
  source 1..20: mol_type = other RNA
aacgggcctggcttgaagtg

SEQ ID NO: 16824 - RNA, 20 nt, synthetic construct
  source 1..20: mol_type = other RNA
gcccgttgatttccaactta

SEQ ID NO: 16825 - RNA, 20 nt, synthetic construct
  source 1..20: mol_type = other RNA
aagttggaaatcaacgggcc

SEQ ID NO: 16826 - RNA, 20 nt, synthetic construct
  source 1..20: mol_type = other RNA
gccataagttggaaatcaac

SEQ ID NO: 16827 - RNA, 20 nt, synthetic construct
  source 1..20: mol_type = other RNA
agccataagttggaaatcaa

SEQ ID NO: 16828 - RNA, 20 nt, synthetic construct
  source 1..20: mol_type = other RNA
tgctgtaggaagccataagt

SEQ ID NO: 16829 - RNA, 20 nt, synthetic construct
  source 1..20: mol_type = other RNA
tatggcttcctacagcagtg

SEQ ID NO: 16830 - RNA, 20 nt, synthetic construct
  source 1..20: mol_type = other RNA
agcagtgtggtcatgaagcc

SEQ ID NO: 16831 - RNA, 20 nt, synthetic construct
  source 1..20: mol_type = other RNA
ggtcatgaagcctggaaaac

SEQ ID NO: 16832 - RNA, 20 nt, synthetic construct
  source 1..20: mol_type = other RNA
agcctggaaaacaggaagat

SEQ ID NO: 16833 - RNA, 20 nt, synthetic construct
  source 1..20: mol_type = other RNA
ctcctatcttcctgttttcc

SEQ ID NO: 16834 - RNA, 20 nt, synthetic construct
  source 1..20: mol_type = other RNA
gaagataggagtgacaaaag

SEQ ID NO: 16835 - RNA, 20 nt, synthetic construct
  source 1..20: mol_type = other RNA
aagataggagtgacaaaaga

SEQ ID NO: 16836 - RNA, 20 nt, synthetic construct
  source 1..20: mol_type = other RNA
aggagtgacaaaagagggac

SEQ ID NO: 16837 - RNA, 20 nt, synthetic construct
  source 1..20: mol_type = other RNA
agagggacaggagtagaatg

SEQ ID NO: 16838 - RNA, 20 nt, synthetic construct
  source 1..20: mol_type = other RNA
acaggagtagaatgaggctt

SEQ ID NO: 16839 - RNA, 20 nt, synthetic construct
  source 1..20: mol_type = other RNA
aaaagatgctcatttcattt

SEQ ID NO: 16840 - RNA, 20 nt, synthetic construct
  source 1..20: mol_type = other RNA
catttcattttggatgacta

SEQ ID NO: 16841 - RNA, 20 nt, synthetic construct
  source 1..20: mol_type = other RNA
cattttggatgactatggca

SEQ ID NO: 16842 - RNA, 20 nt, synthetic construct
  source 1..20: mol_type = other RNA
atgactatggcaaggaagag

SEQ ID NO: 16843 - RNA, 20 nt, synthetic construct
  source 1..20: mol_type = other RNA
actatggcaaggaagagtgg

SEQ ID NO: 16844 - RNA, 20 nt, synthetic construct
  source 1..20: mol_type = other RNA
gactaacagtagcagtagac

SEQ ID NO: 16845 - RNA, 20 nt, synthetic construct
  source 1..20: mol_type = other RNA
gactgtttttatgtattcat

SEQ ID NO: 16846 - RNA, 20 nt, synthetic construct
  source 1..20: mol_type = other RNA
attcattggtttaaattccc

SEQ ID NO: 16847 - RNA, 20 nt, synthetic construct
  source 1..20: mol_type = other RNA
gacatgtttctggagatcca

SEQ ID NO: 16848 - RNA, 20 nt, synthetic construct
  source 1..20: mol_type = other RNA
tgacatgtttctggagatcc

SEQ ID NO: 16849 - RNA, 20 nt, synthetic construct
  source 1..20: mol_type = other RNA
agaaacatgtcactttccac

SEQ ID NO: 16850 - RNA, 20 nt, synthetic construct
  source 1..20: mol_type = other RNA
gaaacatgtcactttccact

SEQ ID NO: 16851 - RNA, 20 nt, synthetic construct
  source 1..20: mol_type = other RNA
aaacatgtcactttccactg

SEQ ID NO: 16852 - RNA, 20 nt, synthetic construct
  source 1..20: mol_type = other RNA
agtggaaagtgacatgtttc

SEQ ID NO: 16853 - RNA, 20 nt, synthetic construct
  source 1..20: mol_type = other RNA
atgacacaaatttcccccag

SEQ ID NO: 16854 - RNA, 20 nt, synthetic construct
  source 1..20: mol_type = other RNA
taacactgagaaaggaggag

SEQ ID NO: 16855 - RNA, 20 nt, synthetic construct
  source 1..20: mol_type = other RNA
ttaacactgagaaaggagga

SEQ ID NO: 16856 - RNA, 20 nt, synthetic construct
  source 1..20: mol_type = other RNA
attaacactgagaaaggagg

SEQ ID NO: 16857 - RNA, 20 nt, synthetic construct
  source 1..20: mol_type = other RNA
gtgattaacactgagaaagg

SEQ ID NO: 16858 - RNA, 20 nt, synthetic construct
  source 1..20: mol_type = other RNA
aaggtgattaacactgagaa

SEQ ID NO: 16859 - RNA, 20 nt, synthetic construct
  source 1..20: mol_type = other RNA
taagtgctaattataggaga

SEQ ID NO: 16860 - RNA, 20 nt, synthetic construct
  source 1..20: mol_type = other RNA
acattttaagtgctaattat

SEQ ID NO: 16861 - RNA, 20 nt, synthetic construct
  source 1..20: mol_type = other RNA
attagcacttaaaatgtcaa

SEQ ID NO: 16862 - RNA, 20 nt, synthetic construct
  source 1..20: mol_type = other RNA
aggagaagaaattaattaac

SEQ ID NO: 16863 - RNA, 20 nt, synthetic construct
  source 1..20: mol_type = other RNA
caggagtatccagtgcagca

SEQ ID NO: 16864 - RNA, 20 nt, synthetic construct
  source 1..20: mol_type = other RNA
atccagtgcagcaaggctct

SEQ ID NO: 16865 - RNA, 20 nt, synthetic construct
  source 1..20: mol_type = other RNA
gtcctagagccttgctgcac

SEQ ID NO: 16866 - RNA, 20 nt, synthetic construct
  source 1..20: mol_type = other RNA
ttaaatattttgagtgcttt

SEQ ID NO: 16867 - RNA, 20 nt, synthetic construct
  source 1..20: mol_type = other RNA
taaatattttgagtgctttt

SEQ ID NO: 16868 - RNA, 20 nt, synthetic construct
  source 1..20: mol_type = other RNA
aaaagcactcaaaatattta

SEQ ID NO: 16869 - RNA, 20 nt, synthetic construct
  source 1..20: mol_type = other RNA
ggatctttcaattagaaggg

SEQ ID NO: 16870 - RNA, 20 nt, synthetic construct
  source 1..20: mol_type = other RNA
taaggatctttcaattagaa

SEQ ID NO: 16871 - RNA, 20 nt, synthetic construct
  source 1..20: mol_type = other RNA
ttaaggatctttcaattaga

SEQ ID NO: 16872 - RNA, 20 nt, synthetic construct
  source 1..20: mol_type = other RNA
cttaactacaccctaagtcc

SEQ ID NO: 16873 - RNA, 20 nt, synthetic construct
  source 1..20: mol_type = other RNA
caggacttagggtgtagtta

SEQ ID NO: 16874 - RNA, 20 nt, synthetic construct
  source 1..20: mol_type = other RNA
acaccctaagtcctggctgg

SEQ ID NO: 16875 - RNA, 20 nt, synthetic construct
  source 1..20: mol_type = other RNA
ctaagtcctggctggtggcc

SEQ ID NO: 16876 - RNA, 20 nt, synthetic construct
  source 1..20: mol_type = other RNA
taagtcctggctggtggcca

SEQ ID NO: 16877 - RNA, 20 nt, synthetic construct
  source 1..20: mol_type = other RNA
aagtcctggctggtggccag

SEQ ID NO: 16878 - RNA, 20 nt, synthetic construct
  source 1..20: mol_type = other RNA
tggccaccagccaggactta

SEQ ID NO: 16879 - RNA, 20 nt, synthetic construct
  source 1..20: mol_type = other RNA
ctggccaccagccaggactt

SEQ ID NO: 16880 - RNA, 20 nt, synthetic construct
  source 1..20: mol_type = other RNA
ctggctggtggccaggggtg

SEQ ID NO: 16881 - RNA, 20 nt, synthetic construct
  source 1..20: mol_type = other RNA
tggctggtggccaggggtgc

SEQ ID NO: 16882 - RNA, 20 nt, synthetic construct
  source 1..20: mol_type = other RNA
ggctggtggccaggggtgcg

SEQ ID NO: 16883 - RNA, 20 nt, synthetic construct
  source 1..20: mol_type = other RNA
cgcacccctggccaccagcc

SEQ ID NO: 16884 - RNA, 20 nt, synthetic construct
  source 1..20: mol_type = other RNA
caggggtgcggggctgagtg

SEQ ID NO: 16885 - RNA, 20 nt, synthetic construct
  source 1..20: mol_type = other RNA
gggtgcggggctgagtgagg

SEQ ID NO: 16886 - RNA, 20 nt, synthetic construct
  source 1..20: mol_type = other RNA
ctcactcagccccgcacccc

SEQ ID NO: 16887 - RNA, 20 nt, synthetic construct
  source 1..20: mol_type = other RNA
gggctgagtgaggcggcgtg

SEQ ID NO: 16888 - RNA, 20 nt, synthetic construct
  source 1..20: mol_type = other RNA
aatcccttcttcaccatcct

SEQ ID NO: 16889 - RNA, 20 nt, synthetic construct
  source 1..20: mol_type = other RNA
atcccttcttcaccatcctt

SEQ ID NO: 16890 - RNA, 20 nt, synthetic construct
  source 1..20: mol_type = other RNA
ttcccaaggatggtgaagaa

SEQ ID NO: 16891 - RNA, 20 nt, synthetic construct
  source 1..20: mol_type = other RNA
tttcccaaggatggtgaaga

SEQ ID NO: 16892 - RNA, 20 nt, synthetic construct
  source 1..20: mol_type = other RNA
ggagggaattttcccaagga

SEQ ID NO: 16893 - RNA, 20 nt, synthetic construct
  source 1..20: mol_type = other RNA
tgggaaaattccctccaaac

SEQ ID NO: 16894 - RNA, 20 nt, synthetic construct
  source 1..20: mol_type = other RNA
gggaaaattccctccaaact

SEQ ID NO: 16895 - RNA, 20 nt, synthetic construct
  source 1..20: mol_type = other RNA
gtttggagggaattttccca

SEQ ID NO: 16896 - RNA, 20 nt, synthetic construct
  source 1..20: mol_type = other RNA
aattccctccaaactgggat

SEQ ID NO: 16897 - RNA, 20 nt, synthetic construct
  source 1..20: mol_type = other RNA
tccctccaaactgggatagg

SEQ ID NO: 16898 - RNA, 20 nt, synthetic construct
  source 1..20: mol_type = other RNA
gccacctatcccagtttgga

SEQ ID NO: 16899 - RNA, 20 nt, synthetic construct
  source 1..20: mol_type = other RNA
tgccacctatcccagtttgg

SEQ ID NO: 16900 - RNA, 20 nt, synthetic construct
  source 1..20: mol_type = other RNA
actgggataggtggcaacag

SEQ ID NO: 16901 - RNA, 20 nt, synthetic construct
  source 1..20: mol_type = other RNA
tgttgccacctatcccagtt

SEQ ID NO: 16902 - RNA, 20 nt, synthetic construct
  source 1..20: mol_type = other RNA
gataggtggcaacagaggtt

SEQ ID NO: 16903 - RNA, 20 nt, synthetic construct
  source 1..20: mol_type = other RNA
tcggaaacagcaagcgtccc

SEQ ID NO: 16904 - RNA, 20 nt, synthetic construct
  source 1..20: mol_type = other RNA
agcgtcccaggctgaatctg

SEQ ID NO: 16905 - RNA, 20 nt, synthetic construct
  source 1..20: mol_type = other RNA
gtcccaggctgaatctgcgg

SEQ ID NO: 16906 - RNA, 20 nt, synthetic construct
  source 1..20: mol_type = other RNA
ccaggctgaatctgcggagg

SEQ ID NO: 16907 - RNA, 20 nt, synthetic construct
  source 1..20: mol_type = other RNA
ctcctccgcagattcagcct

SEQ ID NO: 16908 - RNA, 20 nt, synthetic construct
  source 1..20: mol_type = other RNA
cctcctccgcagattcagcc

SEQ ID NO: 16909 - RNA, 20 nt, synthetic construct
  source 1..20: mol_type = other RNA
gagatgaacctttcctgagc

SEQ ID NO: 16910 - RNA, 20 nt, synthetic construct
  source 1..20: mol_type = other RNA
acgcagtaccagctcaggaa

SEQ ID NO: 16911 - RNA, 20 nt, synthetic construct
  source 1..20: mol_type = other RNA
ctgagctggtactgcgtgcc

SEQ ID NO: 16912 - RNA, 20 nt, synthetic construct
  source 1..20: mol_type = other RNA
ctggcacgcagtaccagctc

SEQ ID NO: 16913 - RNA, 20 nt, synthetic construct
  source 1..20: mol_type = other RNA
gcgtgccaggaactttagct

SEQ ID NO: 16914 - RNA, 20 nt, synthetic construct
  source 1..20: mol_type = other RNA
aaataccgagctaaagttcc

SEQ ID NO: 16915 - RNA, 20 nt, synthetic construct
  source 1..20: mol_type = other RNA
tcggttgtcttacaggattg

SEQ ID NO: 16916 - RNA, 20 nt, synthetic construct
  source 1..20: mol_type = other RNA
catagtatcggttgtcttac

SEQ ID NO: 16917 - RNA, 20 nt, synthetic construct
  source 1..20: mol_type = other RNA
taaaatggagatcatagtat

SEQ ID NO: 16918 - RNA, 20 nt, synthetic construct
  source 1..20: mol_type = other RNA
tgatctccattttacagatg

SEQ ID NO: 16919 - RNA, 20 nt, synthetic construct
  source 1..20: mol_type = other RNA
ttttacagatgaggacattg

SEQ ID NO: 16920 - RNA, 20 nt, synthetic construct
  source 1..20: mol_type = other RNA
caatgtcctcatctgtaaaa

SEQ ID NO: 16921 - RNA, 20 nt, synthetic construct
  source 1..20: mol_type = other RNA
gaggacattgaggctcagcg

SEQ ID NO: 16922 - RNA, 20 nt, synthetic construct
  source 1..20: mol_type = other RNA
agcgtggttgtgacttcctc

SEQ ID NO: 16923 - RNA, 20 nt, synthetic construct
  source 1..20: mol_type = other RNA
ttcagtggctgcgtgacctg

SEQ ID NO: 16924 - RNA, 20 nt, synthetic construct
  source 1..20: mol_type = other RNA
tctttggcgctttcattcag

SEQ ID NO: 16925 - RNA, 20 nt, synthetic construct
  source 1..20: mol_type = other RNA
agcgccaaagattcaaactg

SEQ ID NO: 16926 - RNA, 20 nt, synthetic construct
  source 1..20: mol_type = other RNA
cagacctcagtttgaatctt

SEQ ID NO: 16927 - RNA, 20 nt, synthetic construct
  source 1..20: mol_type = other RNA
tctaaagctttgctctctca

SEQ ID NO: 16928 - RNA, 20 nt, synthetic construct
  source 1..20: mol_type = other RNA
tttgctctctcacggcatcc

SEQ ID NO: 16929 - RNA, 20 nt, synthetic construct
  source 1..20: mol_type = other RNA
gaaggttgaaataggattcc

SEQ ID NO: 16930 - RNA, 20 nt, synthetic construct
  source 1..20: mol_type = other RNA
atcctatttcaaccttcatc

SEQ ID NO: 16931 - RNA, 20 nt, synthetic construct
  source 1..20: mol_type = other RNA
gtccagatgaaggttgaaat

SEQ ID NO: 16932 - RNA, 20 nt, synthetic construct
  source 1..20: mol_type = other RNA
tgggttaagagtccagatga

SEQ ID NO: 16933 - RNA, 20 nt, synthetic construct
  source 1..20: mol_type = other RNA
tagacgcttaggtttgggct

SEQ ID NO: 16934 - RNA, 20 nt, synthetic construct
  source 1..20: mol_type = other RNA
gtagacgcttaggtttgggc

SEQ ID NO: 16935 - RNA, 20 nt, synthetic construct
  source 1..20: mol_type = other RNA
aactgtagacgcttaggttt

SEQ ID NO: 16936 - RNA, 20 nt, synthetic construct
  source 1..20: mol_type = other RNA
aaactgtagacgcttaggtt

SEQ ID NO: 16937 - RNA, 20 nt, synthetic construct
  source 1..20: mol_type = other RNA
tgtcaaaactgtagacgctt

SEQ ID NO: 16938 - RNA, 20 nt, synthetic construct
  source 1..20: mol_type = other RNA
gtctacagttttgacagctg

SEQ ID NO: 16939 - RNA, 20 nt, synthetic construct
  source 1..20: mol_type = other RNA
tacagttttgacagctgagg

SEQ ID NO: 16940 - RNA, 20 nt, synthetic construct
  source 1..20: mol_type = other RNA
acagttttgacagctgaggc

SEQ ID NO: 16941 - RNA, 20 nt, synthetic construct
  source 1..20: mol_type = other RNA
tgacagctgaggcgggagca

SEQ ID NO: 16942 - RNA, 20 nt, synthetic construct
  source 1..20: mol_type = other RNA
gacagctgaggcgggagcac

SEQ ID NO: 16943 - RNA, 20 nt, synthetic construct
  source 1..20: mol_type = other RNA
agctgaggcgggagcacggg

SEQ ID NO: 16944 - RNA, 20 nt, synthetic construct
  source 1..20: mol_type = other RNA
tgaggcgggagcacgggagg

SEQ ID NO: 16945 - RNA, 20 nt, synthetic construct
  source 1..20: mol_type = other RNA
gggagcacgggaggcggagc

SEQ ID NO: 16946 - RNA, 20 nt, synthetic construct
  source 1..20: mol_type = other RNA
agcacgggaggcggagctgg

SEQ ID NO: 16947 - RNA, 20 nt, synthetic construct
  source 1..20: mol_type = other RNA
ggcagcgcagcgccccgccc

SEQ ID NO: 16948 - RNA, 20 nt, synthetic construct
  source 1..20: mol_type = other RNA
ctgatgctggagccggggcg

SEQ ID NO: 16949 - RNA, 20 nt, synthetic construct
  source 1..20: mol_type = other RNA
gctgatgctggagccggggc

SEQ ID NO: 16950 - RNA, 20 nt, synthetic construct
  source 1..20: mol_type = other RNA
ggctgatgctggagccgggg

SEQ ID NO: 16951 - RNA, 20 nt, synthetic construct
  source 1..20: mol_type = other RNA
attggctgatgctggagccg

SEQ ID NO: 16952 - RNA, 20 nt, synthetic construct
  source 1..20: mol_type = other RNA
cattggctgatgctggagcc

SEQ ID NO: 16953 - RNA, 20 nt, synthetic construct
  source 1..20: mol_type = other RNA
ccattggctgatgctggagc

SEQ ID NO: 16954 - RNA, 20 nt, synthetic construct
  source 1..20: mol_type = other RNA
agcatcagccaatggtgacg

SEQ ID NO: 16955 - RNA, 20 nt, synthetic construct
  source 1..20: mol_type = other RNA
gcgtcaccattggctgatgc

SEQ ID NO: 16956 - RNA, 20 nt, synthetic construct
  source 1..20: mol_type = other RNA
tgtgggtgccgcgtcaccat

SEQ ID NO: 16957 - RNA, 20 nt, synthetic construct
  source 1..20: mol_type = other RNA
ctgattgggcgaaaggctgt

SEQ ID NO: 16958 - RNA, 20 nt, synthetic construct
  source 1..20: mol_type = other RNA
gctgattgggcgaaaggctg

SEQ ID NO: 16959 - RNA, 20 nt, synthetic construct
  source 1..20: mol_type = other RNA
gctcaagctgattgggcgaa

SEQ ID NO: 16960 - RNA, 20 nt, synthetic construct
  source 1..20: mol_type = other RNA
gcgggaagctcaagctgatt

SEQ ID NO: 16961 - RNA, 20 nt, synthetic construct
  source 1..20: mol_type = other RNA
ggcgggaagctcaagctgat

SEQ ID NO: 16962 - RNA, 20 nt, synthetic construct
  source 1..20: mol_type = other RNA
gaagagcggcggatggaggc

SEQ ID NO: 16963 - RNA, 20 nt, synthetic construct
  source 1..20: mol_type = other RNA
agaagagcggcggatggagg

SEQ ID NO: 16964 - RNA, 20 nt, synthetic construct
  source 1..20: mol_type = other RNA
cagagaagagcggcggatgg

SEQ ID NO: 16965 - RNA, 20 nt, synthetic construct
  source 1..20: mol_type = other RNA
gggcagagaagagcggcgga

SEQ ID NO: 16966 - RNA, 20 nt, synthetic construct
  source 1..20: mol_type = other RNA
ggcggggcagagaagagcgg

SEQ ID NO: 16967 - RNA, 20 nt, synthetic construct
  source 1..20: mol_type = other RNA
aggggcggggcagagaagag

SEQ ID NO: 16968 - RNA, 20 nt, synthetic construct
  source 1..20: mol_type = other RNA
ccgccccttcgctttccctt

SEQ ID NO: 16969 - RNA, 20 nt, synthetic construct
  source 1..20: mol_type = other RNA
aaagggaaagcgaaggggcg

SEQ ID NO: 16970 - RNA, 20 nt, synthetic construct
  source 1..20: mol_type = other RNA
caaagggaaagcgaaggggc

SEQ ID NO: 16971 - RNA, 20 nt, synthetic construct
  source 1..20: mol_type = other RNA
ccaaagggaaagcgaagggg

SEQ ID NO: 16972 - RNA, 20 nt, synthetic construct
  source 1..20: mol_type = other RNA
gaaccaaagggaaagcgaag

SEQ ID NO: 16973 - RNA, 20 nt, synthetic construct
  source 1..20: mol_type = other RNA
ggaaccaaagggaaagcgaa

SEQ ID NO: 16974 - RNA, 20 nt, synthetic construct
  source 1..20: mol_type = other RNA
tggaaccaaagggaaagcga

SEQ ID NO: 16975 - RNA, 20 nt, synthetic construct
  source 1..20: mol_type = other RNA
tcaagctcggtggaaccaaa

SEQ ID NO: 16976 - RNA, 20 nt, synthetic construct
  source 1..20: mol_type = other RNA
gtcaagctcggtggaaccaa

SEQ ID NO: 16977 - RNA, 20 nt, synthetic construct
  source 1..20: mol_type = other RNA
ttccaccgagcttgacagag

SEQ ID NO: 16978 - RNA, 20 nt, synthetic construct
  source 1..20: mol_type = other RNA
ttccgctctgtcaagctcgg

SEQ ID NO: 16979 - RNA, 20 nt, synthetic construct
  source 1..20: mol_type = other RNA
actttccgctctgtcaagct

SEQ ID NO: 16980 - RNA, 20 nt, synthetic construct
  source 1..20: mol_type = other RNA
gacagagcggaaagtccctt

SEQ ID NO: 16981 - RNA, 20 nt, synthetic construct
  source 1..20: mol_type = other RNA
gagcggaaagtcccttcggc

SEQ ID NO: 16982 - RNA, 20 nt, synthetic construct
  source 1..20: mol_type = other RNA
aaagtcccttcggccggcgc

SEQ ID NO: 16983 - RNA, 20 nt, synthetic construct
  source 1..20: mol_type = other RNA
aagtcccttcggccggcgcc

SEQ ID NO: 16984 - RNA, 20 nt, synthetic construct
  source 1..20: mol_type = other RNA
cccttcggccggcgccgggc

SEQ ID NO: 16985 - RNA, 20 nt, synthetic construct
  source 1..20: mol_type = other RNA
ccagcccggcgccggccgaa

SEQ ID NO: 16986 - RNA, 20 nt, synthetic construct
  source 1..20: mol_type = other RNA
gccagcccggcgccggccga

SEQ ID NO: 16987 - RNA, 20 nt, synthetic construct
  source 1..20: mol_type = other RNA
ggcgccgggctggcagccat

SEQ ID NO: 16988 - RNA, 20 nt, synthetic construct
  source 1..20: mol_type = other RNA
gccgggctggcagccattgg

SEQ ID NO: 16989 - RNA, 20 nt, synthetic construct
  source 1..20: mol_type = other RNA
ggctggcagccattggagga

SEQ ID NO: 16990 - RNA, 20 nt, synthetic construct
  source 1..20: mol_type = other RNA
tcctccaatggctgccagcc

SEQ ID NO: 16991 - RNA, 20 nt, synthetic construct
  source 1..20: mol_type = other RNA
attggaggaaggtctgtcac

SEQ ID NO: 16992 - RNA, 20 nt, synthetic construct
  source 1..20: mol_type = other RNA
ttggaggaaggtctgtcaca

SEQ ID NO: 16993 - RNA, 20 nt, synthetic construct
  source 1..20: mol_type = other RNA
tgtgacagaccttcctccaa

SEQ ID NO: 16994 - RNA, 20 nt, synthetic construct
  source 1..20: mol_type = other RNA
gaggaaggtctgtcacaggg

SEQ ID NO: 16995 - RNA, 20 nt, synthetic construct
  source 1..20: mol_type = other RNA
gtcacagggaggcccaatca

SEQ ID NO: 16996 - RNA, 20 nt, synthetic construct
  source 1..20: mol_type = other RNA
ggcccaatcacggcccgctc

SEQ ID NO: 16997 - RNA, 20 nt, synthetic construct
  source 1..20: mol_type = other RNA
ctcctgagcgggccgtgatt

SEQ ID NO: 16998 - RNA, 20 nt, synthetic construct
  source 1..20: mol_type = other RNA
gctcctgagcgggccgtgat

SEQ ID NO: 16999 - RNA, 20 nt, synthetic construct
  source 1..20: mol_type = other RNA
gcccgctcaggagcgcagct

SEQ ID NO: 17000 - RNA, 20 nt, synthetic construct
  source 1..20: mol_type = other RNA
gccgagctgcgctcctgagc

SEQ ID NO: 17001 - RNA, 20 nt, synthetic construct
  source 1..20: mol_type = other RNA
ggccgagctgcgctcctgag

SEQ ID NO: 17002 - RNA, 20 nt, synthetic construct
  source 1..20: mol_type = other RNA
agcgcagctcggcctacgat

SEQ ID NO: 17003 - RNA, 20 nt, synthetic construct
  source 1..20: mol_type = other RNA
cggcctacgattggctagcg

SEQ ID NO: 17004 - RNA, 20 nt, synthetic construct
  source 1..20: mol_type = other RNA
cctacgattggctagcgcgg

SEQ ID NO: 17005 - RNA, 20 nt, synthetic construct
  source 1..20: mol_type = other RNA
ccgccgcgctagccaatcgt

SEQ ID NO: 17006 - RNA, 20 nt, synthetic construct
  source 1..20: mol_type = other RNA
ggagggagcgggggcggagg

SEQ ID NO: 17007 - RNA, 20 nt, synthetic construct
  source 1..20: mol_type = other RNA
gggagggagcgggggcggag

SEQ ID NO: 17008 - RNA, 20 nt, synthetic construct
  source 1..20: mol_type = other RNA
agggagggagcgggggcgga

SEQ ID NO: 17009 - RNA, 20 nt, synthetic construct
  source 1..20: mol_type = other RNA
gagggagggagcgggggcgg

SEQ ID NO: 17010 - RNA, 20 nt, synthetic construct
  source 1..20: mol_type = other RNA
gaagagggagggagcggggg

SEQ ID NO: 17011 - RNA, 20 nt, synthetic construct
  source 1..20: mol_type = other RNA
agggaagagggagggagcgg

SEQ ID NO: 17012 - RNA, 20 nt, synthetic construct
  source 1..20: mol_type = other RNA
ctccctccctcttccctgtg

SEQ ID NO: 17013 - RNA, 20 nt, synthetic construct
  source 1..20: mol_type = other RNA
acagggaagagggagggagc

SEQ ID NO: 17014 - RNA, 20 nt, synthetic construct
  source 1..20: mol_type = other RNA
cacagggaagagggagggag

SEQ ID NO: 17015 - RNA, 20 nt, synthetic construct
  source 1..20: mol_type = other RNA
tccctcttccctgtgcggtt

SEQ ID NO: 17016 - RNA, 20 nt, synthetic construct
  source 1..20: mol_type = other RNA
aaccgcacagggaagaggga

SEQ ID NO: 17017 - RNA, 20 nt, synthetic construct
  source 1..20: mol_type = other RNA
gaaccgcacagggaagaggg

SEQ ID NO: 17018 - RNA, 20 nt, synthetic construct
  source 1..20: mol_type = other RNA
ttccctgtgcggttcggagg

SEQ ID NO: 17019 - RNA, 20 nt, synthetic construct
  source 1..20: mol_type = other RNA
tccctgtgcggttcggaggc

SEQ ID NO: 17020 - RNA, 20 nt, synthetic construct
  source 1..20: mol_type = other RNA
ccctgtgcggttcggaggcg

SEQ ID NO: 17021 - RNA, 20 nt, synthetic construct
  source 1..20: mol_type = other RNA
gtgcggttcggaggcggggc

SEQ ID NO: 17022 - RNA, 20 nt, synthetic construct
  source 1..20: mol_type = other RNA
ccccgcctccgaaccgcaca

SEQ ID NO: 17023 - RNA, 20 nt, synthetic construct
  source 1..20: mol_type = other RNA
gccccgcctccgaaccgcac

SEQ ID NO: 17024 - RNA, 20 nt, synthetic construct
  source 1..20: mol_type = other RNA
cggttcggaggcggggcagg

SEQ ID NO: 17025 - RNA, 20 nt, synthetic construct
  source 1..20: mol_type = other RNA
ggttcggaggcggggcaggt

SEQ ID NO: 17026 - RNA, 20 nt, synthetic construct
  source 1..20: mol_type = other RNA
gttcggaggcggggcaggtg

SEQ ID NO: 17027 - RNA, 20 nt, synthetic construct
  source 1..20: mol_type = other RNA
ttcggaggcggggcaggtgg

SEQ ID NO: 17028 - RNA, 20 nt, synthetic construct
  source 1..20: mol_type = other RNA
ggaggcggggcaggtggggg

SEQ ID NO: 17029 - RNA, 20 nt, synthetic construct
  source 1..20: mol_type = other RNA
gaggcggggcaggtgggggc

SEQ ID NO: 17030 - RNA, 20 nt, synthetic construct
  source 1..20: mol_type = other RNA
gggcaggtgggggcgggccc

SEQ ID NO: 17031 - RNA, 20 nt, synthetic construct
  source 1..20: mol_type = other RNA
tgggggcgggcccaggtagc

SEQ ID NO: 17032 - RNA, 20 nt, synthetic construct
  source 1..20: mol_type = other RNA
gcgggcccaggtagcaggtt

SEQ ID NO: 17033 - RNA, 20 nt, synthetic construct
  source 1..20: mol_type = other RNA
aggtagcaggtttggctgcg

SEQ ID NO: 17034 - RNA, 20 nt, synthetic construct
  source 1..20: mol_type = other RNA
ggtagcaggtttggctgcgc

SEQ ID NO: 17035 - RNA, 20 nt, synthetic construct
  source 1..20: mol_type = other RNA
cgcagccaaacctgctacct

SEQ ID NO: 17036 - RNA, 20 nt, synthetic construct
  source 1..20: mol_type = other RNA
gcgcagccaaacctgctacc

SEQ ID NO: 17037 - RNA, 20 nt, synthetic construct
  source 1..20: mol_type = other RNA
gctgcgcgggggccgcgcgt

SEQ ID NO: 17038 - RNA, 20 nt, synthetic construct
  source 1..20: mol_type = other RNA
gcgcgggggccgcgcgtcgg

SEQ ID NO: 17039 - RNA, 20 nt, synthetic construct
  source 1..20: mol_type = other RNA
gcgcgtcggaggtaaatact

SEQ ID NO: 17040 - RNA, 20 nt, synthetic construct
  source 1..20: mol_type = other RNA
cgcgtcggaggtaaatacta

SEQ ID NO: 17041 - RNA, 20 nt, synthetic construct
  source 1..20: mol_type = other RNA
tagtatttacctccgacgcg

SEQ ID NO: 17042 - RNA, 20 nt, synthetic construct
  source 1..20: mol_type = other RNA
gtcggaggtaaatactaggg

SEQ ID NO: 17043 - RNA, 20 nt, synthetic construct
  source 1..20: mol_type = other RNA
ggaggtaaatactagggcgg

SEQ ID NO: 17044 - RNA, 20 nt, synthetic construct
  source 1..20: mol_type = other RNA
gaggtaaatactagggcggt

SEQ ID NO: 17045 - RNA, 20 nt, synthetic construct
  source 1..20: mol_type = other RNA
aaatactagggcggtgggtg

SEQ ID NO: 17046 - RNA, 20 nt, synthetic construct
  source 1..20: mol_type = other RNA
aatactagggcggtgggtgt

SEQ ID NO: 17047 - RNA, 20 nt, synthetic construct
  source 1..20: mol_type = other RNA
atactagggcggtgggtgtg

SEQ ID NO: 17048 - RNA, 20 nt, synthetic construct
  source 1..20: mol_type = other RNA
gggcggtgggtgtggggagc

SEQ ID NO: 17049 - RNA, 20 nt, synthetic construct
  source 1..20: mol_type = other RNA
ggcggtgggtgtggggagcc

SEQ ID NO: 17050 - RNA, 20 nt, synthetic construct
  source 1..20: mol_type = other RNA
gcggtgggtgtggggagccg

SEQ ID NO: 17051 - RNA, 20 nt, synthetic construct
  source 1..20: mol_type = other RNA
tgggtgtggggagccggggc

SEQ ID NO: 17052 - RNA, 20 nt, synthetic construct
  source 1..20: mol_type = other RNA
gtggggagccggggccggcc

SEQ ID NO: 17053 - RNA, 20 nt, synthetic construct
  source 1..20: mol_type = other RNA
tggggagccggggccggccc

SEQ ID NO: 17054 - RNA, 20 nt, synthetic construct
  source 1..20: mol_type = other RNA
gccggggccggcccgggacg

SEQ ID NO: 17055 - RNA, 20 nt, synthetic construct
  source 1..20: mol_type = other RNA
ccggggccggcccgggacgc

SEQ ID NO: 17056 - RNA, 20 nt, synthetic construct
  source 1..20: mol_type = other RNA
ggccggcccgggacgcgggc

SEQ ID NO: 17057 - RNA, 20 nt, synthetic construct
  source 1..20: mol_type = other RNA
gccggcccgggacgcgggct

SEQ ID NO: 17058 - RNA, 20 nt, synthetic construct
  source 1..20: mol_type = other RNA
ccggcccgggacgcgggctg

SEQ ID NO: 17059 - RNA, 20 nt, synthetic construct
  source 1..20: mol_type = other RNA
ccccagcccgcgtcccgggc

SEQ ID NO: 17060 - RNA, 20 nt, synthetic construct
  source 1..20: mol_type = other RNA
cgggacgcgggctggggagc

SEQ ID NO: 17061 - RNA, 20 nt, synthetic construct
  source 1..20: mol_type = other RNA
gggacgcgggctggggagcc

SEQ ID NO: 17062 - RNA, 20 nt, synthetic construct
  source 1..20: mol_type = other RNA
ggacgcgggctggggagccg

SEQ ID NO: 17063 - RNA, 20 nt, synthetic construct
  source 1..20: mol_type = other RNA
ggctccccagcccgcgtccc

SEQ ID NO: 17064 - RNA, 20 nt, synthetic construct
  source 1..20: mol_type = other RNA
cggctccccagcccgcgtcc

SEQ ID NO: 17065 - RNA, 20 nt, synthetic construct
  source 1..20: mol_type = other RNA
cgggctggggagccggggcg

SEQ ID NO: 17066 - RNA, 20 nt, synthetic construct
  source 1..20: mol_type = other RNA
gggctggggagccggggcga

SEQ ID NO: 17067 - RNA, 20 nt, synthetic construct
  source 1..20: mol_type = other RNA
ggctggggagccggggcgag

SEQ ID NO: 17068 - RNA, 20 nt, synthetic construct
  source 1..20: mol_type = other RNA
cggggcgtcgcccctcgccc

SEQ ID NO: 17069 - RNA, 20 nt, synthetic construct
  source 1..20: mol_type = other RNA
gggcgacgccccgccgcccg

SEQ ID NO: 17070 - RNA, 20 nt, synthetic construct
  source 1..20: mol_type = other RNA
ttcactaacctcgggcggcg

SEQ ID NO: 17071 - RNA, 20 nt, synthetic construct
  source 1..20: mol_type = other RNA
attcactaacctcgggcggc

SEQ ID NO: 17072 - RNA, 20 nt, synthetic construct
  source 1..20: mol_type = other RNA
cattcactaacctcgggcgg

SEQ ID NO: 17073 - RNA, 20 nt, synthetic construct
  source 1..20: mol_type = other RNA
cccgaggttagtgaatgagc

SEQ ID NO: 17074 - RNA, 20 nt, synthetic construct
  source 1..20: mol_type = other RNA
gctcattcactaacctcggg

SEQ ID NO: 17075 - RNA, 20 nt, synthetic construct
  source 1..20: mol_type = other RNA
gaggttagtgaatgagcggg

SEQ ID NO: 17076 - RNA, 20 nt, synthetic construct
  source 1..20: mol_type = other RNA
cccgctcattcactaacctc

SEQ ID NO: 17077 - RNA, 20 nt, synthetic construct
  source 1..20: mol_type = other RNA
gcccgctcattcactaacct

SEQ ID NO: 17078 - RNA, 20 nt, synthetic construct
  source 1..20: mol_type = other RNA
ttagtgaatgagcgggcggc

SEQ ID NO: 17079 - RNA, 20 nt, synthetic construct
  source 1..20: mol_type = other RNA
gtgaatgagcgggcggctgg

SEQ ID NO: 17080 - RNA, 20 nt, synthetic construct
  source 1..20: mol_type = other RNA
atgagcgggcggctggcggc

SEQ ID NO: 17081 - RNA, 20 nt, synthetic construct
  source 1..20: mol_type = other RNA
agcgggcggctggcggccgg

SEQ ID NO: 17082 - RNA, 20 nt, synthetic construct
  source 1..20: mol_type = other RNA
gcgggcggctggcggccggc

SEQ ID NO: 17083 - RNA, 20 nt, synthetic construct
  source 1..20: mol_type = other RNA
ggcggctggcggccggcggg

SEQ ID NO: 17084 - RNA, 20 nt, synthetic construct
  source 1..20: mol_type = other RNA
gctggcggccggcgggcggc

SEQ ID NO: 17085 - RNA, 20 nt, synthetic construct
  source 1..20: mol_type = other RNA
ggcgggcggccggatcccct

SEQ ID NO: 17086 - RNA, 20 nt, synthetic construct
  source 1..20: mol_type = other RNA
gaggggatccggccgcccgc

SEQ ID NO: 17087 - RNA, 20 nt, synthetic construct
  source 1..20: mol_type = other RNA
atcccctcggcgcagccgcc

SEQ ID NO: 17088 - RNA, 20 nt, synthetic construct
  source 1..20: mol_type = other RNA
gcggctgcgccgaggggatc

SEQ ID NO: 17089 - RNA, 20 nt, synthetic construct
  source 1..20: mol_type = other RNA
cggcgcagccgcctggcctc

SEQ ID NO: 17090 - RNA, 20 nt, synthetic construct
  source 1..20: mol_type = other RNA
ggcgcagccgcctggcctca

SEQ ID NO: 17091 - RNA, 20 nt, synthetic construct
  source 1..20: mol_type = other RNA
gaggccaggcggctgcgccg

SEQ ID NO: 17092 - RNA, 20 nt, synthetic construct
  source 1..20: mol_type = other RNA
ccgcctggcctcagggcgtc

SEQ ID NO: 17093 - RNA, 20 nt, synthetic construct
  source 1..20: mol_type = other RNA
ccggacgccctgaggccagg

SEQ ID NO: 17094 - RNA, 20 nt, synthetic construct
  source 1..20: mol_type = other RNA
gctccggacgccctgaggcc

SEQ ID NO: 17095 - RNA, 20 nt, synthetic construct
  source 1..20: mol_type = other RNA
cagggcgtccggagccgccg

SEQ ID NO: 17096 - RNA, 20 nt, synthetic construct
  source 1..20: mol_type = other RNA
cggcggctccggacgccctg

SEQ ID NO: 17097 - RNA, 20 nt, synthetic construct
  source 1..20: mol_type = other RNA
ggagccgccgcggcgaccat

SEQ ID NO: 17098 - RNA, 20 nt, synthetic construct
  source 1..20: mol_type = other RNA
gagccgccgcggcgaccatc

SEQ ID NO: 17099 - RNA, 20 nt, synthetic construct
  source 1..20: mol_type = other RNA
gatggtcgccgcggcggctc

SEQ ID NO: 17100 - RNA, 20 nt, synthetic construct
  source 1..20: mol_type = other RNA
cgcggcgaccatcgggccct

SEQ ID NO: 17101 - RNA, 20 nt, synthetic construct
  source 1..20: mol_type = other RNA
gggcccgatggtcgccgcgg

SEQ ID NO: 17102 - RNA, 20 nt, synthetic construct
  source 1..20: mol_type = other RNA
cgagggcccgatggtcgccg

SEQ ID NO: 17103 - RNA, 20 nt, synthetic construct
  source 1..20: mol_type = other RNA
gaccatcgggccctcggcgc

SEQ ID NO: 17104 - RNA, 20 nt, synthetic construct
  source 1..20: mol_type = other RNA
ggccggcgccgagggcccga

SEQ ID NO: 17105 - RNA, 20 nt, synthetic construct
  source 1..20: mol_type = other RNA
aactaacgggccggcgccga

SEQ ID NO: 17106 - RNA, 20 nt, synthetic construct
  source 1..20: mol_type = other RNA
caactaacgggccggcgccg

SEQ ID NO: 17107 - RNA, 20 nt, synthetic construct
  source 1..20: mol_type = other RNA
cgccggcccgttagttgccc

SEQ ID NO: 17108 - RNA, 20 nt, synthetic construct
  source 1..20: mol_type = other RNA
ggcccgggcaactaacgggc

SEQ ID NO: 17109 - RNA, 20 nt, synthetic construct
  source 1..20: mol_type = other RNA
ttagttgcccgggcccgagc

SEQ ID NO: 17110 - RNA, 20 nt, synthetic construct
  source 1..20: mol_type = other RNA
ctcgggcccgggcaactaac

SEQ ID NO: 17111 - RNA, 20 nt, synthetic construct
  source 1..20: mol_type = other RNA
gctcgggcccgggcaactaa

SEQ ID NO: 17112 - RNA, 20 nt, synthetic construct
  source 1..20: mol_type = other RNA
ttgcccgggcccgagccggc

SEQ ID NO: 17113 - RNA, 20 nt, synthetic construct
  source 1..20: mol_type = other RNA
tgcccgggcccgagccggcc

SEQ ID NO: 17114 - RNA, 20 nt, synthetic construct
  source 1..20: mol_type = other RNA
gcccgagccggccgggcccg

SEQ ID NO: 17115 - RNA, 20 nt, synthetic construct
  source 1..20: mol_type = other RNA
cccgagccggccgggcccgc

SEQ ID NO: 17116 - RNA, 20 nt, synthetic construct
  source 1..20: mol_type = other RNA
cccgcgggcccggccggctc

SEQ ID NO: 17117 - RNA, 20 nt, synthetic construct
  source 1..20: mol_type = other RNA
acccgcgggcccggccggct

SEQ ID NO: 17118 - RNA, 20 nt, synthetic construct
  source 1..20: mol_type = other RNA
cggcaacccgcgggcccggc

SEQ ID NO: 17119 - RNA, 20 nt, synthetic construct
  source 1..20: mol_type = other RNA
ggctcggcaacccgcgggcc

SEQ ID NO: 17120 - RNA, 20 nt, synthetic construct
  source 1..20: mol_type = other RNA
cagcgggctcggcaacccgc

SEQ ID NO: 17121 - RNA, 20 nt, synthetic construct
  source 1..20: mol_type = other RNA
tcagcgggctcggcaacccg

SEQ ID NO: 17122 - RNA, 20 nt, synthetic construct
  source 1..20: mol_type = other RNA
cgagcccgctgacgtcagcc

SEQ ID NO: 17123 - RNA, 20 nt, synthetic construct
  source 1..20: mol_type = other RNA
gagcccgctgacgtcagccc

SEQ ID NO: 17124 - RNA, 20 nt, synthetic construct
  source 1..20: mol_type = other RNA
cgggctgacgtcagcgggct

SEQ ID NO: 17125 - RNA, 20 nt, synthetic construct
  source 1..20: mol_type = other RNA
aaacccgggctgacgtcagc

SEQ ID NO: 17126 - RNA, 20 nt, synthetic construct
  source 1..20: mol_type = other RNA
gaaacccgggctgacgtcag

SEQ ID NO: 17127 - RNA, 20 nt, synthetic construct
  source 1..20: mol_type = other RNA
cccgggtttcccccccccac

SEQ ID NO: 17128 - RNA, 20 nt, synthetic construct
  source 1..20: mol_type = other RNA
ccgggtttcccccccccacc

SEQ ID NO: 17129 - RNA, 20 nt, synthetic construct
  source 1..20: mol_type = other RNA
cgggtttcccccccccaccg

SEQ ID NO: 17130 - RNA, 20 nt, synthetic construct
  source 1..20: mol_type = other RNA
ccggtgggggggggaaaccc

SEQ ID NO: 17131 - RNA, 20 nt, synthetic construct
  source 1..20: mol_type = other RNA
cccggtgggggggggaaacc

SEQ ID NO: 17132 - RNA, 20 nt, synthetic construct
  source 1..20: mol_type = other RNA
ggggaagccccggtgggggg

SEQ ID NO: 17133 - RNA, 20 nt, synthetic construct
  source 1..20: mol_type = other RNA
tggggaagccccggtggggg

SEQ ID NO: 17134 - RNA, 20 nt, synthetic construct
  source 1..20: mol_type = other RNA
atggggaagccccggtgggg

SEQ ID NO: 17135 - RNA, 20 nt, synthetic construct
  source 1..20: mol_type = other RNA
gatggggaagccccggtggg

SEQ ID NO: 17136 - RNA, 20 nt, synthetic construct
  source 1..20: mol_type = other RNA
ggatggggaagccccggtgg

SEQ ID NO: 17137 - RNA, 20 nt, synthetic construct
  source 1..20: mol_type = other RNA
gggatggggaagccccggtg

SEQ ID NO: 17138 - RNA, 20 nt, synthetic construct
  source 1..20: mol_type = other RNA
ggggatggggaagccccggt

SEQ ID NO: 17139 - RNA, 20 nt, synthetic construct
  source 1..20: mol_type = other RNA
gggggatggggaagccccgg

SEQ ID NO: 17140 - RNA, 20 nt, synthetic construct
  source 1..20: mol_type = other RNA
ctcgggggatggggaagccc

SEQ ID NO: 17141 - RNA, 20 nt, synthetic construct
  source 1..20: mol_type = other RNA
ccccatcccccgaggcttcc

SEQ ID NO: 17142 - RNA, 20 nt, synthetic construct
  source 1..20: mol_type = other RNA
cccatcccccgaggcttccc

SEQ ID NO: 17143 - RNA, 20 nt, synthetic construct
  source 1..20: mol_type = other RNA
atcccccgaggcttcccggg

SEQ ID NO: 17144 - RNA, 20 nt, synthetic construct
  source 1..20: mol_type = other RNA
ccgggaagcctcgggggatg

SEQ ID NO: 17145 - RNA, 20 nt, synthetic construct
  source 1..20: mol_type = other RNA
cccgggaagcctcgggggat

SEQ ID NO: 17146 - RNA, 20 nt, synthetic construct
  source 1..20: mol_type = other RNA
tcccgggaagcctcggggga

SEQ ID NO: 17147 - RNA, 20 nt, synthetic construct
  source 1..20: mol_type = other RNA
gccctcccgggaagcctcgg

SEQ ID NO: 17148 - RNA, 20 nt, synthetic construct
  source 1..20: mol_type = other RNA
agccctcccgggaagcctcg

SEQ ID NO: 17149 - RNA, 20 nt, synthetic construct
  source 1..20: mol_type = other RNA
cagccctcccgggaagcctc

SEQ ID NO: 17150 - RNA, 20 nt, synthetic construct
  source 1..20: mol_type = other RNA
gcagccctcccgggaagcct

SEQ ID NO: 17151 - RNA, 20 nt, synthetic construct
  source 1..20: mol_type = other RNA
tcccgggagggctgcgagtc

SEQ ID NO: 17152 - RNA, 20 nt, synthetic construct
  source 1..20: mol_type = other RNA
cccgggagggctgcgagtcc

SEQ ID NO: 17153 - RNA, 20 nt, synthetic construct
  source 1..20: mol_type = other RNA
ccgggagggctgcgagtccg

SEQ ID NO: 17154 - RNA, 20 nt, synthetic construct
  source 1..20: mol_type = other RNA
cccggactcgcagccctccc

SEQ ID NO: 17155 - RNA, 20 nt, synthetic construct
  source 1..20: mol_type = other RNA
ccccggactcgcagccctcc

SEQ ID NO: 17156 - RNA, 20 nt, synthetic construct
  source 1..20: mol_type = other RNA
ctgcgagtccggggagcgtg

SEQ ID NO: 17157 - RNA, 20 nt, synthetic construct
  source 1..20: mol_type = other RNA
tgcgagtccggggagcgtgc

SEQ ID NO: 17158 - RNA, 20 nt, synthetic construct
  source 1..20: mol_type = other RNA
gcgagtccggggagcgtgcg

SEQ ID NO: 17159 - RNA, 20 nt, synthetic construct
  source 1..20: mol_type = other RNA
tggcgaccccgcacgctccc

SEQ ID NO: 17160 - RNA, 20 nt, synthetic construct
  source 1..20: mol_type = other RNA
gcgtgcggggtcgccaccat

SEQ ID NO: 17161 - RNA, 20 nt, synthetic construct
  source 1..20: mol_type = other RNA
cgtgcggggtcgccaccatc

SEQ ID NO: 17162 - RNA, 20 nt, synthetic construct
  source 1..20: mol_type = other RNA
gccaccatcgggacccccag

SEQ ID NO: 17163 - RNA, 20 nt, synthetic construct
  source 1..20: mol_type = other RNA
tcctctgggggtcccgatgg

SEQ ID NO: 17164 - RNA, 20 nt, synthetic construct
  source 1..20: mol_type = other RNA
tcgggacccccagaggagag

SEQ ID NO: 17165 - RNA, 20 nt, synthetic construct
  source 1..20: mol_type = other RNA
ctctcctctgggggtcccga

SEQ ID NO: 17166 - RNA, 20 nt, synthetic construct
  source 1..20: mol_type = other RNA
cccccagaggagagaggact

SEQ ID NO: 17167 - RNA, 20 nt, synthetic construct
  source 1..20: mol_type = other RNA
ccccagaggagagaggactt

SEQ ID NO: 17168 - RNA, 20 nt, synthetic construct
  source 1..20: mol_type = other RNA
cccagaggagagaggacttg

SEQ ID NO: 17169 - RNA, 20 nt, synthetic construct
  source 1..20: mol_type = other RNA
agaggagagaggacttgggg

SEQ ID NO: 17170 - RNA, 20 nt, synthetic construct
  source 1..20: mol_type = other RNA
cccaagtcctctctcctctg

SEQ ID NO: 17171 - RNA, 20 nt, synthetic construct
  source 1..20: mol_type = other RNA
ccccaagtcctctctcctct

SEQ ID NO: 17172 - RNA, 20 nt, synthetic construct
  source 1..20: mol_type = other RNA
gccccaagtcctctctcctc

SEQ ID NO: 17173 - RNA, 20 nt, synthetic construct
  source 1..20: mol_type = other RNA
gacttggggcgggagccgcg

SEQ ID NO: 17174 - RNA, 20 nt, synthetic construct
  source 1..20: mol_type = other RNA
acttggggcgggagccgcgc

SEQ ID NO: 17175 - RNA, 20 nt, synthetic construct
  source 1..20: mol_type = other RNA
gagggggacagcgtcccgcg

SEQ ID NO: 17176 - RNA, 20 nt, synthetic construct
  source 1..20: mol_type = other RNA
atggggtggggggcgggagg

SEQ ID NO: 17177 - RNA, 20 nt, synthetic construct
  source 1..20: mol_type = other RNA
aatggggtggggggcgggag

SEQ ID NO: 17178 - RNA, 20 nt, synthetic construct
  source 1..20: mol_type = other RNA
aaatggggtggggggcggga

SEQ ID NO: 17179 - RNA, 20 nt, synthetic construct
  source 1..20: mol_type = other RNA
taaatggggtggggggcggg

SEQ ID NO: 17180 - RNA, 20 nt, synthetic construct
  source 1..20: mol_type = other RNA
cccccaccccatttacagat

SEQ ID NO: 17181 - RNA, 20 nt, synthetic construct
  source 1..20: mol_type = other RNA
ccccaccccatttacagatt

SEQ ID NO: 17182 - RNA, 20 nt, synthetic construct
  source 1..20: mol_type = other RNA
caatctgtaaatggggtggg

SEQ ID NO: 17183 - RNA, 20 nt, synthetic construct
  source 1..20: mol_type = other RNA
ccaatctgtaaatggggtgg

SEQ ID NO: 17184 - RNA, 20 nt, synthetic construct
  source 1..20: mol_type = other RNA
cccaatctgtaaatggggtg

SEQ ID NO: 17185 - RNA, 20 nt, synthetic construct
  source 1..20: mol_type = other RNA
tcccaatctgtaaatggggt

SEQ ID NO: 17186 - RNA, 20 nt, synthetic construct
  source 1..20: mol_type = other RNA
ctcccaatctgtaaatgggg

SEQ ID NO: 17187 - RNA, 20 nt, synthetic construct
  source 1..20: mol_type = other RNA
atttacagattgggagactg

SEQ ID NO: 17188 - RNA, 20 nt, synthetic construct
  source 1..20: mol_type = other RNA
agtctcccaatctgtaaatg

SEQ ID NO: 17189 - RNA, 20 nt, synthetic construct
  source 1..20: mol_type = other RNA
cagtctcccaatctgtaaat

SEQ ID NO: 17190 - RNA, 20 nt, synthetic construct
  source 1..20: mol_type = other RNA
tcagtctcccaatctgtaaa

SEQ ID NO: 17191 - RNA, 20 nt, synthetic construct
  source 1..20: mol_type = other RNA
agattgggagactgaggcac

SEQ ID NO: 17192 - RNA, 20 nt, synthetic construct
  source 1..20: mol_type = other RNA
gagactgaggcacaggccgc

SEQ ID NO: 17193 - RNA, 20 nt, synthetic construct
  source 1..20: mol_type = other RNA
actgaggcacaggccgctgg

SEQ ID NO: 17194 - RNA, 20 nt, synthetic construct
  source 1..20: mol_type = other RNA
ctgaggcacaggccgctggc

SEQ ID NO: 17195 - RNA, 20 nt, synthetic construct
  source 1..20: mol_type = other RNA
aggccgctggcgggccccga

SEQ ID NO: 17196 - RNA, 20 nt, synthetic construct
  source 1..20: mol_type = other RNA
ctggcgggccccgacggcca

SEQ ID NO: 17197 - RNA, 20 nt, synthetic construct
  source 1..20: mol_type = other RNA
tggccgtcggggcccgccag

SEQ ID NO: 17198 - RNA, 20 nt, synthetic construct
  source 1..20: mol_type = other RNA
cgggccccgacggccacggt

SEQ ID NO: 17199 - RNA, 20 nt, synthetic construct
  source 1..20: mol_type = other RNA
cgacggccacggttggcctc

SEQ ID NO: 17200 - RNA, 20 nt, synthetic construct
  source 1..20: mol_type = other RNA
gaggccaaccgtggccgtcg

SEQ ID NO: 17201 - RNA, 20 nt, synthetic construct
  source 1..20: mol_type = other RNA
tgaggccaaccgtggccgtc

SEQ ID NO: 17202 - RNA, 20 nt, synthetic construct
  source 1..20: mol_type = other RNA
ctgaggccaaccgtggccgt

SEQ ID NO: 17203 - RNA, 20 nt, synthetic construct
  source 1..20: mol_type = other RNA
cacggttggcctcaggagcc

SEQ ID NO: 17204 - RNA, 20 nt, synthetic construct
  source 1..20: mol_type = other RNA
acggttggcctcaggagccc

SEQ ID NO: 17205 - RNA, 20 nt, synthetic construct
  source 1..20: mol_type = other RNA
cggttggcctcaggagcccg

SEQ ID NO: 17206 - RNA, 20 nt, synthetic construct
  source 1..20: mol_type = other RNA
cgggctcctgaggccaaccg

SEQ ID NO: 17207 - RNA, 20 nt, synthetic construct
  source 1..20: mol_type = other RNA
atcacagccccgggctcctg

SEQ ID NO: 17208 - RNA, 20 nt, synthetic construct
  source 1..20: mol_type = other RNA
tcggtaggaatcacagcccc

SEQ ID NO: 17209 - RNA, 20 nt, synthetic construct
  source 1..20: mol_type = other RNA
gtcggtaggaatcacagccc

SEQ ID NO: 17210 - RNA, 20 nt, synthetic construct
  source 1..20: mol_type = other RNA
gattcctaccgaccgcgccg

SEQ ID NO: 17211 - RNA, 20 nt, synthetic construct
  source 1..20: mol_type = other RNA
attcctaccgaccgcgccgc

SEQ ID NO: 17212 - RNA, 20 nt, synthetic construct
  source 1..20: mol_type = other RNA
ttcctaccgaccgcgccgcg

SEQ ID NO: 17213 - RNA, 20 nt, synthetic construct
  source 1..20: mol_type = other RNA
cgccccgcggcgcggtcggt

SEQ ID NO: 17214 - RNA, 20 nt, synthetic construct
  source 1..20: mol_type = other RNA
cgtacgccccgcggcgcggt

SEQ ID NO: 17215 - RNA, 20 nt, synthetic construct
  source 1..20: mol_type = other RNA
ggtacgtacgccccgcggcg

SEQ ID NO: 17216 - RNA, 20 nt, synthetic construct
  source 1..20: mol_type = other RNA
cgatcggtacgtacgccccg

SEQ ID NO: 17217 - RNA, 20 nt, synthetic construct
  source 1..20: mol_type = other RNA
gtacgtaccgatcgattttg

SEQ ID NO: 17218 - RNA, 20 nt, synthetic construct
  source 1..20: mol_type = other RNA
tacgtaccgatcgattttgc

SEQ ID NO: 17219 - RNA, 20 nt, synthetic construct
  source 1..20: mol_type = other RNA
ccgatcgattttgcgggtgt

SEQ ID NO: 17220 - RNA, 20 nt, synthetic construct
  source 1..20: mol_type = other RNA
atcgattttgcgggtgttgg

SEQ ID NO: 17221 - RNA, 20 nt, synthetic construct
  source 1..20: mol_type = other RNA
ccaacacccgcaaaatcgat

SEQ ID NO: 17222 - RNA, 20 nt, synthetic construct
  source 1..20: mol_type = other RNA
ggtgttggtggctcccgtcc

SEQ ID NO: 17223 - RNA, 20 nt, synthetic construct
  source 1..20: mol_type = other RNA
tggtggctcccgtccaggaa

SEQ ID NO: 17224 - RNA, 20 nt, synthetic construct
  source 1..20: mol_type = other RNA
tcccgtccaggaatggcagt

SEQ ID NO: 17225 - RNA, 20 nt, synthetic construct
  source 1..20: mol_type = other RNA
cccgtccaggaatggcagtc

SEQ ID NO: 17226 - RNA, 20 nt, synthetic construct
  source 1..20: mol_type = other RNA
ccgtccaggaatggcagtcg

SEQ ID NO: 17227 - RNA, 20 nt, synthetic construct
  source 1..20: mol_type = other RNA
cccgactgccattcctggac

SEQ ID NO: 17228 - RNA, 20 nt, synthetic construct
  source 1..20: mol_type = other RNA
ccccgactgccattcctgga

SEQ ID NO: 17229 - RNA, 20 nt, synthetic construct
  source 1..20: mol_type = other RNA
aggaatggcagtcggggttc

SEQ ID NO: 17230 - RNA, 20 nt, synthetic construct
  source 1..20: mol_type = other RNA
agaaccccgactgccattcc

SEQ ID NO: 17231 - RNA, 20 nt, synthetic construct
  source 1..20: mol_type = other RNA
cggggttctggccttgttaa

SEQ ID NO: 17232 - RNA, 20 nt, synthetic construct
  source 1..20: mol_type = other RNA
agcagaacacgccattaaca

SEQ ID NO: 17233 - RNA, 20 nt, synthetic construct
  source 1..20: mol_type = other RNA
ctttcagtttccccctttct

SEQ ID NO: 17234 - RNA, 20 nt, synthetic construct
  source 1..20: mol_type = other RNA
tttcagtttccccctttcta

SEQ ID NO: 17235 - RNA, 20 nt, synthetic construct
  source 1..20: mol_type = other RNA
gtttccccctttctagggtg

SEQ ID NO: 17236 - RNA, 20 nt, synthetic construct
  source 1..20: mol_type = other RNA
ccccctttctagggtgagga

SEQ ID NO: 17237 - RNA, 20 nt, synthetic construct
  source 1..20: mol_type = other RNA
ccatcctcaccctagaaagg

SEQ ID NO: 17238 - RNA, 20 nt, synthetic construct
  source 1..20: mol_type = other RNA
accatcctcaccctagaaag

SEQ ID NO: 17239 - RNA, 20 nt, synthetic construct
  source 1..20: mol_type = other RNA
aaccatcctcaccctagaaa

SEQ ID NO: 17240 - RNA, 20 nt, synthetic construct
  source 1..20: mol_type = other RNA
gaaccatcctcaccctagaa

SEQ ID NO: 17241 - RNA, 20 nt, synthetic construct
  source 1..20: mol_type = other RNA
gatggttctacacagccacc

SEQ ID NO: 17242 - RNA, 20 nt, synthetic construct
  source 1..20: mol_type = other RNA
cccggagttccttagttgaa

SEQ ID NO: 17243 - RNA, 20 nt, synthetic construct
  source 1..20: mol_type = other RNA
ttcaactaaggaactccggg

SEQ ID NO: 17244 - RNA, 20 nt, synthetic construct
  source 1..20: mol_type = other RNA
cctttcaactaaggaactcc

SEQ ID NO: 17245 - RNA, 20 nt, synthetic construct
  source 1..20: mol_type = other RNA
acctttcaactaaggaactc

SEQ ID NO: 17246 - RNA, 20 nt, synthetic construct
  source 1..20: mol_type = other RNA
cagggcgcacctttcaacta

SEQ ID NO: 17247 - RNA, 20 nt, synthetic construct
  source 1..20: mol_type = other RNA
aaggtgcgccctgctgtgac

SEQ ID NO: 17248 - RNA, 20 nt, synthetic construct
  source 1..20: mol_type = other RNA
aaagaatacctgtcacagca

SEQ ID NO: 17249 - RNA, 20 nt, synthetic construct
  source 1..20: mol_type = other RNA
gaaagaatacctgtcacagc

SEQ ID NO: 17250 - RNA, 20 nt, synthetic construct
  source 1..20: mol_type = other RNA
ttctttcatgttaacaatcg

SEQ ID NO: 17251 - RNA, 20 nt, synthetic construct
  source 1..20: mol_type = other RNA
tctttcatgttaacaatcga

SEQ ID NO: 17252 - RNA, 20 nt, synthetic construct
  source 1..20: mol_type = other RNA
ctttcatgttaacaatcgag

SEQ ID NO: 17253 - RNA, 20 nt, synthetic construct
  source 1..20: mol_type = other RNA
tttcatgttaacaatcgagg

SEQ ID NO: 17254 - RNA, 20 nt, synthetic construct
  source 1..20: mol_type = other RNA
ttcatgttaacaatcgaggg

SEQ ID NO: 17255 - RNA, 20 nt, synthetic construct
  source 1..20: mol_type = other RNA
atgttaacaatcgagggggg

SEQ ID NO: 17256 - RNA, 20 nt, synthetic construct
  source 1..20: mol_type = other RNA
tgttaacaatcgaggggggt

SEQ ID NO: 17257 - RNA, 20 nt, synthetic construct
  source 1..20: mol_type = other RNA
gttaacaatcgaggggggtg

SEQ ID NO: 17258 - RNA, 20 nt, synthetic construct
  source 1..20: mol_type = other RNA
ttaacaatcgaggggggtgg

SEQ ID NO: 17259 - RNA, 20 nt, synthetic construct
  source 1..20: mol_type = other RNA
taacaatcgaggggggtggg

SEQ ID NO: 17260 - RNA, 20 nt, synthetic construct
  source 1..20: mol_type = other RNA
cgaggggggtggggggcgaa

SEQ ID NO: 17261 - RNA, 20 nt, synthetic construct
  source 1..20: mol_type = other RNA
gaggggggtggggggcgaat

SEQ ID NO: 17262 - RNA, 20 nt, synthetic construct
  source 1..20: mol_type = other RNA
aggggggtggggggcgaatg

SEQ ID NO: 17263 - RNA, 20 nt, synthetic construct
  source 1..20: mol_type = other RNA
ggggggtggggggcgaatgg

SEQ ID NO: 17264 - RNA, 20 nt, synthetic construct
  source 1..20: mol_type = other RNA
gggggtggggggcgaatggg

SEQ ID NO: 17265 - RNA, 20 nt, synthetic construct
  source 1..20: mol_type = other RNA
ggtggggggcgaatgggggg

SEQ ID NO: 17266 - RNA, 20 nt, synthetic construct
  source 1..20: mol_type = other RNA
gtggggggcgaatggggggc

SEQ ID NO: 17267 - RNA, 20 nt, synthetic construct
  source 1..20: mol_type = other RNA
tggggggcgaatggggggcg

SEQ ID NO: 17268 - RNA, 20 nt, synthetic construct
  source 1..20: mol_type = other RNA
ggggggcgaatggggggcgg

SEQ ID NO: 17269 - RNA, 20 nt, synthetic construct
  source 1..20: mol_type = other RNA
ggcgaagtcatgaaatcttc

SEQ ID NO: 17270 - RNA, 20 nt, synthetic construct
  source 1..20: mol_type = other RNA
gtcatgaaatcttcaggaga

SEQ ID NO: 17271 - RNA, 20 nt, synthetic construct
  source 1..20: mol_type = other RNA
tcaggagatggtgttgagtt

SEQ ID NO: 17272 - RNA, 20 nt, synthetic construct
  source 1..20: mol_type = other RNA
tgttgagtttggtactcagc

SEQ ID NO: 17273 - RNA, 20 nt, synthetic construct
  source 1..20: mol_type = other RNA
gttgagtttggtactcagct

SEQ ID NO: 17274 - RNA, 20 nt, synthetic construct
  source 1..20: mol_type = other RNA
atcaggttatattgttcata

SEQ ID NO: 17275 - RNA, 20 nt, synthetic construct
  source 1..20: mol_type = other RNA
tttctgattctcaagttatc

SEQ ID NO: 17276 - RNA, 20 nt, synthetic construct
  source 1..20: mol_type = other RNA
cagaaaaacactgcatcttc

SEQ ID NO: 17277 - RNA, 20 nt, synthetic construct
  source 1..20: mol_type = other RNA
tagctacagaaaactaacaa

SEQ ID NO: 17278 - RNA, 20 nt, synthetic construct
  source 1..20: mol_type = other RNA
atatgttgcctttcagaatg

SEQ ID NO: 17279 - RNA, 20 nt, synthetic construct
  source 1..20: mol_type = other RNA
tacaattaccacattctgaa

SEQ ID NO: 17280 - RNA, 20 nt, synthetic construct
  source 1..20: mol_type = other RNA
aagacaatggaaagatgatc

SEQ ID NO: 17281 - RNA, 20 nt, synthetic construct
  source 1..20: mol_type = other RNA
tcaattttccatgaagacaa

SEQ ID NO: 17282 - RNA, 20 nt, synthetic construct
  source 1..20: mol_type = other RNA
gtgccttccaactctcgtct

SEQ ID NO: 17283 - RNA, 20 nt, synthetic construct
  source 1..20: mol_type = other RNA
caaccaagacgagagttgga

SEQ ID NO: 17284 - RNA, 20 nt, synthetic construct
  source 1..20: mol_type = other RNA
cattcaaccaagacgagagt

SEQ ID NO: 17285 - RNA, 20 nt, synthetic construct
  source 1..20: mol_type = other RNA
ggtctggattctgagtaaag

SEQ ID NO: 17286 - RNA, 20 nt, synthetic construct
  source 1..20: mol_type = other RNA
tggtctggattctgagtaaa

SEQ ID NO: 17287 - RNA, 20 nt, synthetic construct
  source 1..20: mol_type = other RNA
atggtctggattctgagtaa

SEQ ID NO: 17288 - RNA, 20 nt, synthetic construct
  source 1..20: mol_type = other RNA
atctgagcttgttgatggtc

SEQ ID NO: 17289 - RNA, 20 nt, synthetic construct
  source 1..20: mol_type = other RNA
tggttatctgagcttgttga

SEQ ID NO: 17290 - RNA, 20 nt, synthetic construct
  source 1..20: mol_type = other RNA
catagatttgaaaacatttc

SEQ ID NO: 17291 - RNA, 20 nt, synthetic construct
  source 1..20: mol_type = other RNA
ctgatgaaggagaacagttc

SEQ ID NO: 17292 - RNA, 20 nt, synthetic construct
  source 1..20: mol_type = other RNA
tccttcatcagcgtccttaa

SEQ ID NO: 17293 - RNA, 20 nt, synthetic construct
  source 1..20: mol_type = other RNA
catcagcgtccttaaaggaa

SEQ ID NO: 17294 - RNA, 20 nt, synthetic construct
  source 1..20: mol_type = other RNA
tcctttaaggacgctgatga

SEQ ID NO: 17295 - RNA, 20 nt, synthetic construct
  source 1..20: mol_type = other RNA
atttgtgtgtatgtgtttac

SEQ ID NO: 17296 - RNA, 20 nt, synthetic construct
  source 1..20: mol_type = other RNA
tttatttttgctttttcact

SEQ ID NO: 17297 - RNA, 20 nt, synthetic construct
  source 1..20: mol_type = other RNA
tttcctttctttttacagca

SEQ ID NO: 17298 - RNA, 20 nt, synthetic construct
  source 1..20: mol_type = other RNA
tgtccatgctgtaaaaagaa

SEQ ID NO: 17299 - RNA, 20 nt, synthetic construct
  source 1..20: mol_type = other RNA
acgttgctgaaaacatgctt

SEQ ID NO: 17300 - RNA, 20 nt, synthetic construct
  source 1..20: mol_type = other RNA
cgttgctgaaaacatgcttt

SEQ ID NO: 17301 - RNA, 20 nt, synthetic construct
  source 1..20: mol_type = other RNA
aaagcatgttttcagcaacg

SEQ ID NO: 17302 - RNA, 20 nt, synthetic construct
  source 1..20: mol_type = other RNA
gccactgaatttatcttttg

SEQ ID NO: 17303 - RNA, 20 nt, synthetic construct
  source 1..20: mol_type = other RNA
accgcaaaagataaattcag

SEQ ID NO: 17304 - RNA, 20 nt, synthetic construct
  source 1..20: mol_type = other RNA
caaaatactaattcaaaaaa

SEQ ID NO: 17305 - RNA, 20 nt, synthetic construct
  source 1..20: mol_type = other RNA
tcaaaatactaattcaaaaa

SEQ ID NO: 17306 - RNA, 20 nt, synthetic construct
  source 1..20: mol_type = other RNA
gttaatatcacaatgagttc

SEQ ID NO: 17307 - RNA, 20 nt, synthetic construct
  source 1..20: mol_type = other RNA
tcacaatgagttcaggctta

SEQ ID NO: 17308 - RNA, 20 nt, synthetic construct
  source 1..20: mol_type = other RNA
agggtgaagtgactttttct

SEQ ID NO: 17309 - RNA, 20 nt, synthetic construct
  source 1..20: mol_type = other RNA
aaaagtcacttcaccctact

SEQ ID NO: 17310 - RNA, 20 nt, synthetic construct
  source 1..20: mol_type = other RNA
cttcaccctactgggaagag

SEQ ID NO: 17311 - RNA, 20 nt, synthetic construct
  source 1..20: mol_type = other RNA
aaaatccgctcttcccagta

SEQ ID NO: 17312 - RNA, 20 nt, synthetic construct
  source 1..20: mol_type = other RNA
aaaaatccgctcttcccagt

SEQ ID NO: 17313 - RNA, 20 nt, synthetic construct
  source 1..20: mol_type = other RNA
aaagctccttaaagtaccga

SEQ ID NO: 17314 - RNA, 20 nt, synthetic construct
  source 1..20: mol_type = other RNA
aagctccttaaagtaccgaa

SEQ ID NO: 17315 - RNA, 20 nt, synthetic construct
  source 1..20: mol_type = other RNA
aaagtaccgaagggaagtat

SEQ ID NO: 17316 - RNA, 20 nt, synthetic construct
  source 1..20: mol_type = other RNA
tacttcccttcggtacttta

SEQ ID NO: 17317 - RNA, 20 nt, synthetic construct
  source 1..20: mol_type = other RNA
tactgtcctatacttccctt

SEQ ID NO: 17318 - RNA, 20 nt, synthetic construct
  source 1..20: mol_type = other RNA
gtatattcaagatcgttctg

SEQ ID NO: 17319 - RNA, 20 nt, synthetic construct
  source 1..20: mol_type = other RNA
tatattcaagatcgttctgt

SEQ ID NO: 17320 - RNA, 20 nt, synthetic construct
  source 1..20: mol_type = other RNA
atattcaagatcgttctgtg

SEQ ID NO: 17321 - RNA, 20 nt, synthetic construct
  source 1..20: mol_type = other RNA
atcgttctgtggggcattca

SEQ ID NO: 17322 - RNA, 20 nt, synthetic construct
  source 1..20: mol_type = other RNA
tcaaggattccttctgcaaa

SEQ ID NO: 17323 - RNA, 20 nt, synthetic construct
  source 1..20: mol_type = other RNA
tttttcttgccttttgcaga

SEQ ID NO: 17324 - RNA, 20 nt, synthetic construct
  source 1..20: mol_type = other RNA
aaaggcaagaaaaatcagat

SEQ ID NO: 17325 - RNA, 20 nt, synthetic construct
  source 1..20: mol_type = other RNA
tcaacaaagagaactgcatg

SEQ ID NO: 17326 - RNA, 20 nt, synthetic construct
  source 1..20: mol_type = other RNA
agttctctttgttgatgaaa

SEQ ID NO: 17327 - RNA, 20 nt, synthetic construct
  source 1..20: mol_type = other RNA
aaagttcacagagttacttt

SEQ ID NO: 17328 - RNA, 20 nt, synthetic construct
  source 1..20: mol_type = other RNA
tttggcaattaccaattgtg

SEQ ID NO: 17329 - RNA, 20 nt, synthetic construct
  source 1..20: mol_type = other RNA
caattaccaattgtgaggag

SEQ ID NO: 17330 - RNA, 20 nt, synthetic construct
  source 1..20: mol_type = other RNA
gctgaacctctcctcacaat

SEQ ID NO: 17331 - RNA, 20 nt, synthetic construct
  source 1..20: mol_type = other RNA
gtctgtttctgtttttaaac

SEQ ID NO: 17332 - RNA, 20 nt, synthetic construct
  source 1..20: mol_type = other RNA
aacagaaacagactaagtaa

SEQ ID NO: 17333 - RNA, 20 nt, synthetic construct
  source 1..20: mol_type = other RNA
taaaggcctccaaatagacg

SEQ ID NO: 17334 - RNA, 20 nt, synthetic construct
  source 1..20: mol_type = other RNA
aaaggcctccaaatagacgt

SEQ ID NO: 17335 - RNA, 20 nt, synthetic construct
  source 1..20: mol_type = other RNA
gacagcccacgtctatttgg

SEQ ID NO: 17336 - RNA, 20 nt, synthetic construct
  source 1..20: mol_type = other RNA
caggacagcccacgtctatt

SEQ ID NO: 17337 - RNA, 20 nt, synthetic construct
  source 1..20: mol_type = other RNA
gtgaaagtacagctgagatc

SEQ ID NO: 17338 - RNA, 20 nt, synthetic construct
  source 1..20: mol_type = other RNA
tgaaagtacagctgagatct

SEQ ID NO: 17339 - RNA, 20 nt, synthetic construct
  source 1..20: mol_type = other RNA
gaaagtacagctgagatctg

SEQ ID NO: 17340 - RNA, 20 nt, synthetic construct
  source 1..20: mol_type = other RNA
tctggggaagaaaaatttcc

SEQ ID NO: 17341 - RNA, 20 nt, synthetic construct
  source 1..20: mol_type = other RNA
cctggagttgtacgcttcag

SEQ ID NO: 17342 - RNA, 20 nt, synthetic construct
  source 1..20: mol_type = other RNA
cctctgaagcgtacaactcc

SEQ ID NO: 17343 - RNA, 20 nt, synthetic construct
  source 1..20: mol_type = other RNA
gaggacccctgttagcagag

SEQ ID NO: 17344 - RNA, 20 nt, synthetic construct
  source 1..20: mol_type = other RNA
actgtcctctctgctaacag

SEQ ID NO: 17345 - RNA, 20 nt, synthetic construct
  source 1..20: mol_type = other RNA
gactgtcctctctgctaaca

SEQ ID NO: 17346 - RNA, 20 nt, synthetic construct
  source 1..20: mol_type = other RNA
agactgtcctctctgctaac

SEQ ID NO: 17347 - RNA, 20 nt, synthetic construct
  source 1..20: mol_type = other RNA
acagtctccggaatattctt

SEQ ID NO: 17348 - RNA, 20 nt, synthetic construct
  source 1..20: mol_type = other RNA
ttcaactccaaagaatattc

SEQ ID NO: 17349 - RNA, 20 nt, synthetic construct
  source 1..20: mol_type = other RNA
attctttggagttgaattgc

SEQ ID NO: 17350 - RNA, 20 nt, synthetic construct
  source 1..20: mol_type = other RNA
aaacaaacacactactaaaa

SEQ ID NO: 17351 - RNA, 20 nt, synthetic construct
  source 1..20: mol_type = other RNA
gaaaatttatttcgtattta

SEQ ID NO: 17352 - RNA, 20 nt, synthetic construct
  source 1..20: mol_type = other RNA
ggatttcaggaaaatcactc

SEQ ID NO: 17353 - RNA, 20 nt, synthetic construct
  source 1..20: mol_type = other RNA
gggttcactctagggatttc

SEQ ID NO: 17354 - RNA, 20 nt, synthetic construct
  source 1..20: mol_type = other RNA
agagtgaaccccttttccta

SEQ ID NO: 17355 - RNA, 20 nt, synthetic construct
  source 1..20: mol_type = other RNA
aggaaaaggggttcactcta

SEQ ID NO: 17356 - RNA, 20 nt, synthetic construct
  source 1..20: mol_type = other RNA
taggaaaaggggttcactct

SEQ ID NO: 17357 - RNA, 20 nt, synthetic construct
  source 1..20: mol_type = other RNA
aagacgatccataggaaaag

SEQ ID NO: 17358 - RNA, 20 nt, synthetic construct
  source 1..20: mol_type = other RNA
aaagacgatccataggaaaa

SEQ ID NO: 17359 - RNA, 20 nt, synthetic construct
  source 1..20: mol_type = other RNA
gaaagacgatccataggaaa

SEQ ID NO: 17360 - RNA, 20 nt, synthetic construct
  source 1..20: mol_type = other RNA
gatatagaaagacgatccat

SEQ ID NO: 17361 - RNA, 20 nt, synthetic construct
  source 1..20: mol_type = other RNA
tcccttctctcttaaaaact

SEQ ID NO: 17362 - RNA, 20 nt, synthetic construct
  source 1..20: mol_type = other RNA
tcctagtttttaagagagaa

SEQ ID NO: 17363 - RNA, 20 nt, synthetic construct
  source 1..20: mol_type = other RNA
ttcctagtttttaagagaga

SEQ ID NO: 17364 - RNA, 20 nt, synthetic construct
  source 1..20: mol_type = other RNA
aaaaactaggaagaaggtcg

SEQ ID NO: 17365 - RNA, 20 nt, synthetic construct
  source 1..20: mol_type = other RNA
taggaagaaggtcgtggtca

SEQ ID NO: 17366 - RNA, 20 nt, synthetic construct
  source 1..20: mol_type = other RNA
cgtggtcaaggtttcactga

SEQ ID NO: 17367 - RNA, 20 nt, synthetic construct
  source 1..20: mol_type = other RNA
gtggtcaaggtttcactgac

SEQ ID NO: 17368 - RNA, 20 nt, synthetic construct
  source 1..20: mol_type = other RNA
tggtcaaggtttcactgacg

SEQ ID NO: 17369 - RNA, 20 nt, synthetic construct
  source 1..20: mol_type = other RNA
ttcactgacggggtgtacca

SEQ ID NO: 17370 - RNA, 20 nt, synthetic construct
  source 1..20: mol_type = other RNA
tcactgacggggtgtaccaa

SEQ ID NO: 17371 - RNA, 20 nt, synthetic construct
  source 1..20: mol_type = other RNA
actgaaaaagctgtttccct

SEQ ID NO: 17372 - RNA, 20 nt, synthetic construct
  source 1..20: mol_type = other RNA
tttcagtgtgatgaagattg

SEQ ID NO: 17373 - RNA, 20 nt, synthetic construct
  source 1..20: mol_type = other RNA
ttgtggcgtgtttgttgcat

SEQ ID NO: 17374 - RNA, 20 nt, synthetic construct
  source 1..20: mol_type = other RNA
agaagatgatgacactgcat

SEQ ID NO: 17375 - RNA, 20 nt, synthetic construct
  source 1..20: mol_type = other RNA
gcattggaaagtgattacgc

SEQ ID NO: 17376 - RNA, 20 nt, synthetic construct
  source 1..20: mol_type = other RNA
gaaagtgattacgcaggtcc

SEQ ID NO: 17377 - RNA, 20 nt, synthetic construct
  source 1..20: mol_type = other RNA
aaagtgattacgcaggtcct

SEQ ID NO: 17378 - RNA, 20 nt, synthetic construct
  source 1..20: mol_type = other RNA
aagtgattacgcaggtcctg

SEQ ID NO: 17379 - RNA, 20 nt, synthetic construct
  source 1..20: mol_type = other RNA
aggtcctggggacacaatgc

SEQ ID NO: 17380 - RNA, 20 nt, synthetic construct
  source 1..20: mol_type = other RNA
tcgacctgcattgtgtcccc

SEQ ID NO: 17381 - RNA, 20 nt, synthetic construct
  source 1..20: mol_type = other RNA
gcaggtcgaacttcctcctt

SEQ ID NO: 17382 - RNA, 20 nt, synthetic construct
  source 1..20: mol_type = other RNA
ctggagtttatttccaaagg

SEQ ID NO: 17383 - RNA, 20 nt, synthetic construct
  source 1..20: mol_type = other RNA
actctggagtttatttccaa

SEQ ID NO: 17384 - RNA, 20 nt, synthetic construct
  source 1..20: mol_type = other RNA
aaactccagagtttctttga

SEQ ID NO: 17385 - RNA, 20 nt, synthetic construct
  source 1..20: mol_type = other RNA
tccagagtttctttgaaggt

SEQ ID NO: 17386 - RNA, 20 nt, synthetic construct
  source 1..20: mol_type = other RNA
tccaaccttcaaagaaactc

SEQ ID NO: 17387 - RNA, 20 nt, synthetic construct
  source 1..20: mol_type = other RNA
gttggagaaacaatagaatc

SEQ ID NO: 17388 - RNA, 20 nt, synthetic construct
  source 1..20: mol_type = other RNA
atattctgtgatgttttgcc

SEQ ID NO: 17389 - RNA, 20 nt, synthetic construct
  source 1..20: mol_type = other RNA
ttgccaggaaaagaaagctt

SEQ ID NO: 17390 - RNA, 20 nt, synthetic construct
  source 1..20: mol_type = other RNA
tatcctaagctttcttttcc

SEQ ID NO: 17391 - RNA, 20 nt, synthetic construct
  source 1..20: mol_type = other RNA
gaaagcttaggatattttgt

SEQ ID NO: 17392 - RNA, 20 nt, synthetic construct
  source 1..20: mol_type = other RNA
cttaggatattttgttggtg

SEQ ID NO: 17393 - RNA, 20 nt, synthetic construct
  source 1..20: mol_type = other RNA
atattttgttggtgtggaca

SEQ ID NO: 17394 - RNA, 20 nt, synthetic construct
  source 1..20: mol_type = other RNA
tggacatggtaagaaaattt

SEQ ID NO: 17395 - RNA, 20 nt, synthetic construct
  source 1..20: mol_type = other RNA
tttaccaatgtaaaatattt

SEQ ID NO: 17396 - RNA, 20 nt, synthetic construct
  source 1..20: mol_type = other RNA
accaatgtaaaatattttgg

SEQ ID NO: 17397 - RNA, 20 nt, synthetic construct
  source 1..20: mol_type = other RNA
tcctccaaaatattttacat

SEQ ID NO: 17398 - RNA, 20 nt, synthetic construct
  source 1..20: mol_type = other RNA
atattttggaggattcttta

SEQ ID NO: 17399 - RNA, 20 nt, synthetic construct
  source 1..20: mol_type = other RNA
tccacatttacatttcattg

SEQ ID NO: 17400 - RNA, 20 nt, synthetic construct
  source 1..20: mol_type = other RNA
acatttacatttcattgagg

SEQ ID NO: 17401 - RNA, 20 nt, synthetic construct
  source 1..20: mol_type = other RNA
tcctcaatgaaatgtaaatg

SEQ ID NO: 17402 - RNA, 20 nt, synthetic construct
  source 1..20: mol_type = other RNA
atgtttattatttaatttct

SEQ ID NO: 17403 - RNA, 20 nt, synthetic construct
  source 1..20: mol_type = other RNA
aatttctaggataaccctat

SEQ ID NO: 17404 - RNA, 20 nt, synthetic construct
  source 1..20: mol_type = other RNA
aggataaccctattggcaac

SEQ ID NO: 17405 - RNA, 20 nt, synthetic construct
  source 1..20: mol_type = other RNA
ggataaccctattggcaact

SEQ ID NO: 17406 - RNA, 20 nt, synthetic construct
  source 1..20: mol_type = other RNA
aaccctattggcaactggga

SEQ ID NO: 17407 - RNA, 20 nt, synthetic construct
  source 1..20: mol_type = other RNA
ttccatcccagttgccaata

SEQ ID NO: 17408 - RNA, 20 nt, synthetic construct
  source 1..20: mol_type = other RNA
cttccatcccagttgccaat

SEQ ID NO: 17409 - RNA, 20 nt, synthetic construct
  source 1..20: mol_type = other RNA
aactgggatggaagatttga

SEQ ID NO: 17410 - RNA, 20 nt, synthetic construct
  source 1..20: mol_type = other RNA
cacatcaatgatatcatccc

SEQ ID NO: 17411 - RNA, 20 nt, synthetic construct
  source 1..20: mol_type = other RNA
aaaacaaagaaaacatacct

SEQ ID NO: 17412 - RNA, 20 nt, synthetic construct
  source 1..20: mol_type = other RNA
taaaacaaagaaaacatacc

SEQ ID NO: 17413 - RNA, 20 nt, synthetic construct
  source 1..20: mol_type = other RNA
ctttgttttatacatttata

SEQ ID NO: 17414 - RNA, 20 nt, synthetic construct
  source 1..20: mol_type = other RNA
ttttttatatcaatatgttt

SEQ ID NO: 17415 - RNA, 20 nt, synthetic construct
  source 1..20: mol_type = other RNA
tttttatatcaatatgtttt

SEQ ID NO: 17416 - RNA, 20 nt, synthetic construct
  source 1..20: mol_type = other RNA
ttttatatcaatatgttttg

SEQ ID NO: 17417 - RNA, 20 nt, synthetic construct
  source 1..20: mol_type = other RNA
tttatatcaatatgttttgg

SEQ ID NO: 17418 - RNA, 20 nt, synthetic construct
  source 1..20: mol_type = other RNA
tcaatatgttttgggggaac

SEQ ID NO: 17419 - RNA, 20 nt, synthetic construct
  source 1..20: mol_type = other RNA
atatgttttgggggaacagg

SEQ ID NO: 17420 - RNA, 20 nt, synthetic construct
  source 1..20: mol_type = other RNA
ttgggggaacaggtggtgtt

SEQ ID NO: 17421 - RNA, 20 nt, synthetic construct
  source 1..20: mol_type = other RNA
acaggtggtgtttggttaca

SEQ ID NO: 17422 - RNA, 20 nt, synthetic construct
  source 1..20: mol_type = other RNA
tacatggataagttctttcg

SEQ ID NO: 17423 - RNA, 20 nt, synthetic construct
  source 1..20: mol_type = other RNA
aagacttttcttaaaaaaag

SEQ ID NO: 17424 - RNA, 20 nt, synthetic construct
  source 1..20: mol_type = other RNA
atttttacattttaaacaca

SEQ ID NO: 17425 - RNA, 20 nt, synthetic construct
  source 1..20: mol_type = other RNA
gaggacagaaagaaagaaat

SEQ ID NO: 17426 - RNA, 20 nt, synthetic construct
  source 1..20: mol_type = other RNA
ttctgtcctcaaatccactg

SEQ ID NO: 17427 - RNA, 20 nt, synthetic construct
  source 1..20: mol_type = other RNA
tctgtcctcaaatccactgt

SEQ ID NO: 17428 - RNA, 20 nt, synthetic construct
  source 1..20: mol_type = other RNA
tatcacccacagtggatttg

SEQ ID NO: 17429 - RNA, 20 nt, synthetic construct
  source 1..20: mol_type = other RNA
aaaaacgatatcacccacag

SEQ ID NO: 17430 - RNA, 20 nt, synthetic construct
  source 1..20: mol_type = other RNA
tgctgacacacagctttatc

SEQ ID NO: 17431 - RNA, 20 nt, synthetic construct
  source 1..20: mol_type = other RNA
atgactcctaagtgtcgtgt

SEQ ID NO: 17432 - RNA, 20 nt, synthetic construct
  source 1..20: mol_type = other RNA
aagtgtcgtgttggactcca

SEQ ID NO: 17433 - RNA, 20 nt, synthetic construct
  source 1..20: mol_type = other RNA
tggagtccaacacgacactt

SEQ ID NO: 17434 - RNA, 20 nt, synthetic construct
  source 1..20: mol_type = other RNA
aaaattcaacaatacatccg

SEQ ID NO: 17435 - RNA, 20 nt, synthetic construct
  source 1..20: mol_type = other RNA
tgtattgttgaatttttcaa

SEQ ID NO: 17436 - RNA, 20 nt, synthetic construct
  source 1..20: mol_type = other RNA
tgatcaagggaatgtagaag

SEQ ID NO: 17437 - RNA, 20 nt, synthetic construct
  source 1..20: mol_type = other RNA
cattcccttgatcagtattt

SEQ ID NO: 17438 - RNA, 20 nt, synthetic construct
  source 1..20: mol_type = other RNA
tactcctaaatactgatcaa

SEQ ID NO: 17439 - RNA, 20 nt, synthetic construct
  source 1..20: mol_type = other RNA
atactcctaaatactgatca

SEQ ID NO: 17440 - RNA, 20 nt, synthetic construct
  source 1..20: mol_type = other RNA
ctaaaaattctgcctttttg

SEQ ID NO: 17441 - RNA, 20 nt, synthetic construct
  source 1..20: mol_type = other RNA
ttctgcctttttgtggaaag

SEQ ID NO: 17442 - RNA, 20 nt, synthetic construct
  source 1..20: mol_type = other RNA
tctgcctttttgtggaaaga

SEQ ID NO: 17443 - RNA, 20 nt, synthetic construct
  source 1..20: mol_type = other RNA
aaaaccctctttccacaaaa

SEQ ID NO: 17444 - RNA, 20 nt, synthetic construct
  source 1..20: mol_type = other RNA
attcttatagaagagaaaca

SEQ ID NO: 17445 - RNA, 20 nt, synthetic construct
  source 1..20: mol_type = other RNA
agcatgttttttaaagataa

SEQ ID NO: 17446 - RNA, 20 nt, synthetic construct
  source 1..20: mol_type = other RNA
tgtttcagagagtgtgacgc

SEQ ID NO: 17447 - RNA, 20 nt, synthetic construct
  source 1..20: mol_type = other RNA
cagagagtgtgacgcaggaa

SEQ ID NO: 17448 - RNA, 20 nt, synthetic construct
  source 1..20: mol_type = other RNA
agagtgtgacgcaggaaagg

SEQ ID NO: 17449 - RNA, 20 nt, synthetic construct
  source 1..20: mol_type = other RNA
gacataaaggcaagtttggg

SEQ ID NO: 17450 - RNA, 20 nt, synthetic construct
  source 1..20: mol_type = other RNA
aaacttgcctttatgtcaag

SEQ ID NO: 17451 - RNA, 20 nt, synthetic construct
  source 1..20: mol_type = other RNA
cttgacataaaggcaagttt

SEQ ID NO: 17452 - RNA, 20 nt, synthetic construct
  source 1..20: mol_type = other RNA
tcttgacataaaggcaagtt

SEQ ID NO: 17453 - RNA, 20 nt, synthetic construct
  source 1..20: mol_type = other RNA
gcctttatgtcaagaggtgt

SEQ ID NO: 17454 - RNA, 20 nt, synthetic construct
  source 1..20: mol_type = other RNA
cctttatgtcaagaggtgtt

SEQ ID NO: 17455 - RNA, 20 nt, synthetic construct
  source 1..20: mol_type = other RNA
ctttatgtcaagaggtgttg

SEQ ID NO: 17456 - RNA, 20 nt, synthetic construct
  source 1..20: mol_type = other RNA
cccaacacctcttgacataa

SEQ ID NO: 17457 - RNA, 20 nt, synthetic construct
  source 1..20: mol_type = other RNA
tcaagaggtgttggggacaa

SEQ ID NO: 17458 - RNA, 20 nt, synthetic construct
  source 1..20: mol_type = other RNA
atccagtcataataaaccaa

SEQ ID NO: 17459 - RNA, 20 nt, synthetic construct
  source 1..20: mol_type = other RNA
agcctttggtttattatgac

SEQ ID NO: 17460 - RNA, 20 nt, synthetic construct
  source 1..20: mol_type = other RNA
taaaccaaaggctacaggta

SEQ ID NO: 17461 - RNA, 20 nt, synthetic construct
  source 1..20: mol_type = other RNA
taatccatacctgtagcctt

SEQ ID NO: 17462 - RNA, 20 nt, synthetic construct
  source 1..20: mol_type = other RNA
ggcattatgcaaattactaa

SEQ ID NO: 17463 - RNA, 20 nt, synthetic construct
  source 1..20: mol_type = other RNA
ttttaatgctatggcaagtt

SEQ ID NO: 17464 - RNA, 20 nt, synthetic construct
  source 1..20: mol_type = other RNA
tataatcttttttaatgcta

SEQ ID NO: 17465 - RNA, 20 nt, synthetic construct
  source 1..20: mol_type = other RNA
gaaacttttcttgttcctat

SEQ ID NO: 17466 - RNA, 20 nt, synthetic construct
  source 1..20: mol_type = other RNA
ataggatctacctcagaccc

SEQ ID NO: 17467 - RNA, 20 nt, synthetic construct
  source 1..20: mol_type = other RNA
gggtctgaggtagatcctat

SEQ ID NO: 17468 - RNA, 20 nt, synthetic construct
  source 1..20: mol_type = other RNA
gtttctatttccagggtctg

SEQ ID NO: 17469 - RNA, 20 nt, synthetic construct
  source 1..20: mol_type = other RNA
cagatctgtttctatttcca

SEQ ID NO: 17470 - RNA, 20 nt, synthetic construct
  source 1..20: mol_type = other RNA
tcagatctgtttctatttcc

SEQ ID NO: 17471 - RNA, 20 nt, synthetic construct
  source 1..20: mol_type = other RNA
gaattattttataccttaaa

SEQ ID NO: 17472 - RNA, 20 nt, synthetic construct
  source 1..20: mol_type = other RNA
aattattttataccttaaat

SEQ ID NO: 17473 - RNA, 20 nt, synthetic construct
  source 1..20: mol_type = other RNA
gtcaacagaagacccattta

SEQ ID NO: 17474 - RNA, 20 nt, synthetic construct
  source 1..20: mol_type = other RNA
aatccaaatcaaaaaataca

SEQ ID NO: 17475 - RNA, 20 nt, synthetic construct
  source 1..20: mol_type = other RNA
gtattttttgatttggattg

SEQ ID NO: 17476 - RNA, 20 nt, synthetic construct
  source 1..20: mol_type = other RNA
gtaccatgtattttttgatt

SEQ ID NO: 17477 - RNA, 20 nt, synthetic construct
  source 1..20: mol_type = other RNA
aatacatggtacattgatga

SEQ ID NO: 17478 - RNA, 20 nt, synthetic construct
  source 1..20: mol_type = other RNA
ctctgatgagttagaaagaa

SEQ ID NO: 17479 - RNA, 20 nt, synthetic construct
  source 1..20: mol_type = other RNA
tctaactcatcagagaaaaa

SEQ ID NO: 17480 - RNA, 20 nt, synthetic construct
  source 1..20: mol_type = other RNA
atatcaatatttgtagtttt

SEQ ID NO: 17481 - RNA, 20 nt, synthetic construct
  source 1..20: mol_type = other RNA
ctattaatagcagggaggtc

SEQ ID NO: 17482 - RNA, 20 nt, synthetic construct
  source 1..20: mol_type = other RNA
ttaatagcagggaggtcagg

SEQ ID NO: 17483 - RNA, 20 nt, synthetic construct
  source 1..20: mol_type = other RNA
taatagcagggaggtcaggt

SEQ ID NO: 17484 - RNA, 20 nt, synthetic construct
  source 1..20: mol_type = other RNA
agggaggtcaggtgggcagt

SEQ ID NO: 17485 - RNA, 20 nt, synthetic construct
  source 1..20: mol_type = other RNA
ttgaatacatttctgtaatt

SEQ ID NO: 17486 - RNA, 20 nt, synthetic construct
  source 1..20: mol_type = other RNA
taattacagaaatgtattca

SEQ ID NO: 17487 - RNA, 20 nt, synthetic construct
  source 1..20: mol_type = other RNA
tctctgtaagagattttgca

SEQ ID NO: 17488 - RNA, 20 nt, synthetic construct
  source 1..20: mol_type = other RNA
atctctgtaagagattttgc

SEQ ID NO: 17489 - RNA, 20 nt, synthetic construct
  source 1..20: mol_type = other RNA
gctggagtggtggtgaagaa

SEQ ID NO: 17490 - RNA, 20 nt, synthetic construct
  source 1..20: mol_type = other RNA
acaggaggaggctggagtgg

SEQ ID NO: 17491 - RNA, 20 nt, synthetic construct
  source 1..20: mol_type = other RNA
ttcacaggaggaggctggag

SEQ ID NO: 17492 - RNA, 20 nt, synthetic construct
  source 1..20: mol_type = other RNA
gtgagttcacaggaggaggc

SEQ ID NO: 17493 - RNA, 20 nt, synthetic construct
  source 1..20: mol_type = other RNA
gtcagtgagttcacaggagg

SEQ ID NO: 17494 - RNA, 20 nt, synthetic construct
  source 1..20: mol_type = other RNA
gtggtcagtgagttcacagg

SEQ ID NO: 17495 - RNA, 20 nt, synthetic construct
  source 1..20: mol_type = other RNA
tcggtggtcagtgagttcac

SEQ ID NO: 17496 - RNA, 20 nt, synthetic construct
  source 1..20: mol_type = other RNA
agagtggaatctgttctcgg

SEQ ID NO: 17497 - RNA, 20 nt, synthetic construct
  source 1..20: mol_type = other RNA
taaagagtggaatctgttct

SEQ ID NO: 17498 - RNA, 20 nt, synthetic construct
  source 1..20: mol_type = other RNA
tgagactgaatggtaaagag

SEQ ID NO: 17499 - RNA, 20 nt, synthetic construct
  source 1..20: mol_type = other RNA
ggcatcttggtgagactgaa

SEQ ID NO: 17500 - RNA, 20 nt, synthetic construct
  source 1..20: mol_type = other RNA
accaagatgcccaataccaa

SEQ ID NO: 17501 - RNA, 20 nt, synthetic construct
  source 1..20: mol_type = other RNA
tccattggtattgggcatct

SEQ ID NO: 17502 - RNA, 20 nt, synthetic construct
  source 1..20: mol_type = other RNA
cccaataccaatggaagtat

SEQ ID NO: 17503 - RNA, 20 nt, synthetic construct
  source 1..20: mol_type = other RNA
ccaatacttccattggtatt

SEQ ID NO: 17504 - RNA, 20 nt, synthetic construct
  source 1..20: mol_type = other RNA
gccaatacttccattggtat

SEQ ID NO: 17505 - RNA, 20 nt, synthetic construct
  source 1..20: mol_type = other RNA
actgtggccaatacttccat

SEQ ID NO: 17506 - RNA, 20 nt, synthetic construct
  source 1..20: mol_type = other RNA
ctgacagagaaagtggactg

SEQ ID NO: 17507 - RNA, 20 nt, synthetic construct
  source 1..20: mol_type = other RNA
gactgggctgacagagaaag

SEQ ID NO: 17508 - RNA, 20 nt, synthetic construct
  source 1..20: mol_type = other RNA
tctgtcagcccagtctgtaa

SEQ ID NO: 17509 - RNA, 20 nt, synthetic construct
  source 1..20: mol_type = other RNA
tagctcttccattacagact

SEQ ID NO: 17510 - RNA, 20 nt, synthetic construct
  source 1..20: mol_type = other RNA
ttagctcttccattacagac

SEQ ID NO: 17511 - RNA, 20 nt, synthetic construct
  source 1..20: mol_type = other RNA
cgtccaagagagtccaccct

SEQ ID NO: 17512 - RNA, 20 nt, synthetic construct
  source 1..20: mol_type = other RNA
aagggtggactctcttggac

SEQ ID NO: 17513 - RNA, 20 nt, synthetic construct
  source 1..20: mol_type = other RNA
caagggtggactctcttgga

SEQ ID NO: 17514 - RNA, 20 nt, synthetic construct
  source 1..20: mol_type = other RNA
tggccaagggtggactctct

SEQ ID NO: 17515 - RNA, 20 nt, synthetic construct
  source 1..20: mol_type = other RNA
ccacccttggccatgcctcc

SEQ ID NO: 17516 - RNA, 20 nt, synthetic construct
  source 1..20: mol_type = other RNA
cacccttggccatgcctcct

SEQ ID NO: 17517 - RNA, 20 nt, synthetic construct
  source 1..20: mol_type = other RNA
ccaggaggcatggccaaggg

SEQ ID NO: 17518 - RNA, 20 nt, synthetic construct
  source 1..20: mol_type = other RNA
ttcccaggaggcatggccaa

SEQ ID NO: 17519 - RNA, 20 nt, synthetic construct
  source 1..20: mol_type = other RNA
gttcccaggaggcatggcca

SEQ ID NO: 17520 - RNA, 20 nt, synthetic construct
  source 1..20: mol_type = other RNA
atgcctcctgggaactcaca

SEQ ID NO: 17521 - RNA, 20 nt, synthetic construct
  source 1..20: mol_type = other RNA
atgtgagttcccaggaggca

SEQ ID NO: 17522 - RNA, 20 nt, synthetic construct
  source 1..20: mol_type = other RNA
agaccatgtgagttcccagg

SEQ ID NO: 17523 - RNA, 20 nt, synthetic construct
  source 1..20: mol_type = other RNA
gaactcacatggtctagaag

SEQ ID NO: 17524 - RNA, 20 nt, synthetic construct
  source 1..20: mol_type = other RNA
aactcacatggtctagaagt

SEQ ID NO: 17525 - RNA, 20 nt, synthetic construct
  source 1..20: mol_type = other RNA
tggtctagaagtgggctcat

SEQ ID NO: 17526 - RNA, 20 nt, synthetic construct
  source 1..20: mol_type = other RNA
gggctcattggctgaagtta

SEQ ID NO: 17527 - RNA, 20 nt, synthetic construct
  source 1..20: mol_type = other RNA
aaggagaaccctcctttcta

SEQ ID NO: 17528 - RNA, 20 nt, synthetic construct
  source 1..20: mol_type = other RNA
aggagaaccctcctttctat

SEQ ID NO: 17529 - RNA, 20 nt, synthetic construct
  source 1..20: mol_type = other RNA
ggagaaccctcctttctatg

SEQ ID NO: 17530 - RNA, 20 nt, synthetic construct
  source 1..20: mol_type = other RNA
ctttctatggggtaatccgt

SEQ ID NO: 17531 - RNA, 20 nt, synthetic construct
  source 1..20: mol_type = other RNA
cggattaccccatagaaagg

SEQ ID NO: 17532 - RNA, 20 nt, synthetic construct
  source 1..20: mol_type = other RNA
caacggattaccccatagaa

SEQ ID NO: 17533 - RNA, 20 nt, synthetic construct
  source 1..20: mol_type = other RNA
tatggggtaatccgttggat

SEQ ID NO: 17534 - RNA, 20 nt, synthetic construct
  source 1..20: mol_type = other RNA
cgttggatcggtcagccacc

SEQ ID NO: 17535 - RNA, 20 nt, synthetic construct
  source 1..20: mol_type = other RNA
ctggtggctgaccgatccaa

SEQ ID NO: 17536 - RNA, 20 nt, synthetic construct
  source 1..20: mol_type = other RNA
agcacttcattcagtcctgg

SEQ ID NO: 17537 - RNA, 20 nt, synthetic construct
  source 1..20: mol_type = other RNA
ggactgaatgaagtgctcgc

SEQ ID NO: 17538 - RNA, 20 nt, synthetic construct
  source 1..20: mol_type = other RNA
gcgagcacttcattcagtcc

SEQ ID NO: 17539 - RNA, 20 nt, synthetic construct
  source 1..20: mol_type = other RNA
gaatgaagtgctcgctggac

SEQ ID NO: 17540 - RNA, 20 nt, synthetic construct
  source 1..20: mol_type = other RNA
agtgctcgctggactggaac

SEQ ID NO: 17541 - RNA, 20 nt, synthetic construct
  source 1..20: mol_type = other RNA
agaaaaaaattgaaattttt

SEQ ID NO: 17542 - RNA, 20 nt, synthetic construct
  source 1..20: mol_type = other RNA
gagaaaaaaattgaaatttt

SEQ ID NO: 17543 - RNA, 20 nt, synthetic construct
  source 1..20: mol_type = other RNA
tttcaatttttttctctgtg

SEQ ID NO: 17544 - RNA, 20 nt, synthetic construct
  source 1..20: mol_type = other RNA
ttgtcaaaaagcatataata

SEQ ID NO: 17545 - RNA, 20 nt, synthetic construct
  source 1..20: mol_type = other RNA
tttgtcaaaaagcatataat

SEQ ID NO: 17546 - RNA, 20 nt, synthetic construct
  source 1..20: mol_type = other RNA
cgaagagggagtggtgagaa

SEQ ID NO: 17547 - RNA, 20 nt, synthetic construct
  source 1..20: mol_type = other RNA
gaagagggagtggtgagaaa

SEQ ID NO: 17548 - RNA, 20 nt, synthetic construct
  source 1..20: mol_type = other RNA
agaaagggtatactagaaac

SEQ ID NO: 17549 - RNA, 20 nt, synthetic construct
  source 1..20: mol_type = other RNA
agatagtatacaaagaacta

SEQ ID NO: 17550 - RNA, 20 nt, synthetic construct
  source 1..20: mol_type = other RNA
ctttgtatactatctctgta

SEQ ID NO: 17551 - RNA, 20 nt, synthetic construct
  source 1..20: mol_type = other RNA
tatactatctctgtaaggca

SEQ ID NO: 17552 - RNA, 20 nt, synthetic construct
  source 1..20: mol_type = other RNA
tattgaagcatttctttttc

SEQ ID NO: 17553 - RNA, 20 nt, synthetic construct
  source 1..20: mol_type = other RNA
tttcaggaagatgagtgtgc

SEQ ID NO: 17554 - RNA, 20 nt, synthetic construct
  source 1..20: mol_type = other RNA
agatgagtgtgcaggctgta

SEQ ID NO: 17555 - RNA, 20 nt, synthetic construct
  source 1..20: mol_type = other RNA
gagtgtgcaggctgtacgga

SEQ ID NO: 17556 - RNA, 20 nt, synthetic construct
  source 1..20: mol_type = other RNA
tgtacggatggaaccttcag

SEQ ID NO: 17557 - RNA, 20 nt, synthetic construct
  source 1..20: mol_type = other RNA
atggaaccttcagaggcact

SEQ ID NO: 17558 - RNA, 20 nt, synthetic construct
  source 1..20: mol_type = other RNA
gaaataccgagtgcctctga

SEQ ID NO: 17559 - RNA, 20 nt, synthetic construct
  source 1..20: mol_type = other RNA
tttcacctgtgccctgaaga

SEQ ID NO: 17560 - RNA, 20 nt, synthetic construct
  source 1..20: mol_type = other RNA
cagcgccttcttcagggcac

SEQ ID NO: 17561 - RNA, 20 nt, synthetic construct
  source 1..20: mol_type = other RNA
cacaaacagcgccttcttca

SEQ ID NO: 17562 - RNA, 20 nt, synthetic construct
  source 1..20: mol_type = other RNA
tcacaaacagcgccttcttc

SEQ ID NO: 17563 - RNA, 20 nt, synthetic construct
  source 1..20: mol_type = other RNA
ttgtgaaactgaagagctgc

SEQ ID NO: 17564 - RNA, 20 nt, synthetic construct
  source 1..20: mol_type = other RNA
agagctgcaggcctgactct

SEQ ID NO: 17565 - RNA, 20 nt, synthetic construct
  source 1..20: mol_type = other RNA
aatgatgcaaacctagagtc

SEQ ID NO: 17566 - RNA, 20 nt, synthetic construct
  source 1..20: mol_type = other RNA
taggtttgcatcattgcagc

SEQ ID NO: 17567 - RNA, 20 nt, synthetic construct
  source 1..20: mol_type = other RNA
cgctcaatctgattggaaac

SEQ ID NO: 17568 - RNA, 20 nt, synthetic construct
  source 1..20: mol_type = other RNA
gttacagcgctcaatctgat

SEQ ID NO: 17569 - RNA, 20 nt, synthetic construct
  source 1..20: mol_type = other RNA
attgagcgctgtaactcttt

SEQ ID NO: 17570 - RNA, 20 nt, synthetic construct
  source 1..20: mol_type = other RNA
gctgtaactctttaggtatt

SEQ ID NO: 17571 - RNA, 20 nt, synthetic construct
  source 1..20: mol_type = other RNA
tttttgtttacttaacaacc

SEQ ID NO: 17572 - RNA, 20 nt, synthetic construct
  source 1..20: mol_type = other RNA
attagaattagagtcattcc

SEQ ID NO: 17573 - RNA, 20 nt, synthetic construct
  source 1..20: mol_type = other RNA
atctcatatcatgttatatt

SEQ ID NO: 17574 - RNA, 20 nt, synthetic construct
  source 1..20: mol_type = other RNA
tatcatgttatattaggtga

SEQ ID NO: 17575 - RNA, 20 nt, synthetic construct
  source 1..20: mol_type = other RNA
ttaaaatgaaaaaatattta

SEQ ID NO: 17576 - RNA, 20 nt, synthetic construct
  source 1..20: mol_type = other RNA
taaaatgaaaaaatatttat

SEQ ID NO: 17577 - RNA, 20 nt, synthetic construct
  source 1..20: mol_type = other RNA
aaaaaaatcttttcagcatt

SEQ ID NO: 17578 - RNA, 20 nt, synthetic construct
  source 1..20: mol_type = other RNA
aaaatcttttcagcatttgg

SEQ ID NO: 17579 - RNA, 20 nt, synthetic construct
  source 1..20: mol_type = other RNA
agaaaatactccaccaaaaa

SEQ ID NO: 17580 - RNA, 20 nt, synthetic construct
  source 1..20: mol_type = other RNA
ccaccaaaaatggaaaaaga

SEQ ID NO: 17581 - RNA, 20 nt, synthetic construct
  source 1..20: mol_type = other RNA
aaaaatggaaaaagaaggct

SEQ ID NO: 17582 - RNA, 20 nt, synthetic construct
  source 1..20: mol_type = other RNA
aagccttctttttccatttt

SEQ ID NO: 17583 - RNA, 20 nt, synthetic construct
  source 1..20: mol_type = other RNA
gaaggcttggagataatgat

SEQ ID NO: 17584 - RNA, 20 nt, synthetic construct
  source 1..20: mol_type = other RNA
aaggcttggagataatgatt

SEQ ID NO: 17585 - RNA, 20 nt, synthetic construct
  source 1..20: mol_type = other RNA
ataatgattgggaagaagaa

SEQ ID NO: 17586 - RNA, 20 nt, synthetic construct
  source 1..20: mol_type = other RNA
tgggaagaagaaaggcatcc

SEQ ID NO: 17587 - RNA, 20 nt, synthetic construct
  source 1..20: mol_type = other RNA
gggaagaagaaaggcatcca

SEQ ID NO: 17588 - RNA, 20 nt, synthetic construct
  source 1..20: mol_type = other RNA
aacaagaattgtaatgaccc

SEQ ID NO: 17589 - RNA, 20 nt, synthetic construct
  source 1..20: mol_type = other RNA
acttagactcaaccttattc

SEQ ID NO: 17590 - RNA, 20 nt, synthetic construct
  source 1..20: mol_type = other RNA
tttttaaacttaccagaata

SEQ ID NO: 17591 - RNA, 20 nt, synthetic construct
  source 1..20: mol_type = other RNA
aagtttaaaaagaatgcaat

SEQ ID NO: 17592 - RNA, 20 nt, synthetic construct
  source 1..20: mol_type = other RNA
taggtatagatagtgccatg

SEQ ID NO: 17593 - RNA, 20 nt, synthetic construct
  source 1..20: mol_type = other RNA
tatagatagtgccatgaggc

SEQ ID NO: 17594 - RNA, 20 nt, synthetic construct
  source 1..20: mol_type = other RNA
atagatagtgccatgaggca

SEQ ID NO: 17595 - RNA, 20 nt, synthetic construct
  source 1..20: mol_type = other RNA
catgaggcagggacacatac

SEQ ID NO: 17596 - RNA, 20 nt, synthetic construct
  source 1..20: mol_type = other RNA
cggtatgtgtccctgcctca

SEQ ID NO: 17597 - RNA, 20 nt, synthetic construct
  source 1..20: mol_type = other RNA
acgcacacacacacacacac

SEQ ID NO: 17598 - RNA, 20 nt, synthetic construct
  source 1..20: mol_type = other RNA
agaggaaaataagtaaagtc

SEQ ID NO: 17599 - RNA, 20 nt, synthetic construct
  source 1..20: mol_type = other RNA
atttttaacagaattagaag

SEQ ID NO: 17600 - RNA, 20 nt, synthetic construct
  source 1..20: mol_type = other RNA
aaataagctgcaaaagaaaa

SEQ ID NO: 17601 - RNA, 20 nt, synthetic construct
  source 1..20: mol_type = other RNA
atttgcttttagttctgttc

SEQ ID NO: 17602 - RNA, 20 nt, synthetic construct
  source 1..20: mol_type = other RNA
tctacatcgttcttttcttt

SEQ ID NO: 17603 - RNA, 20 nt, synthetic construct
  source 1..20: mol_type = other RNA
ttctacatcgttcttttctt

SEQ ID NO: 17604 - RNA, 20 nt, synthetic construct
  source 1..20: mol_type = other RNA
gtgaaacccaagagctactg

SEQ ID NO: 17605 - RNA, 20 nt, synthetic construct
  source 1..20: mol_type = other RNA
ttctgtcctcagtagctctt

SEQ ID NO: 17606 - RNA, 20 nt, synthetic construct
  source 1..20: mol_type = other RNA
tttctgtcctcagtagctct

SEQ ID NO: 17607 - RNA, 20 nt, synthetic construct
  source 1..20: mol_type = other RNA
ttttctacttacattctcag

SEQ ID NO: 17608 - RNA, 20 nt, synthetic construct
  source 1..20: mol_type = other RNA
attgctattttgcctttaca

SEQ ID NO: 17609 - RNA, 20 nt, synthetic construct
  source 1..20: mol_type = other RNA
gcaaatagaacaccatgtaa

SEQ ID NO: 17610 - RNA, 20 nt, synthetic construct
  source 1..20: mol_type = other RNA
gtgttctatttgctgttttc

SEQ ID NO: 17611 - RNA, 20 nt, synthetic construct
  source 1..20: mol_type = other RNA
tgtcttcatgtaataagaga

SEQ ID NO: 17612 - RNA, 20 nt, synthetic construct
  source 1..20: mol_type = other RNA
gtcttcatgtaataagagat

SEQ ID NO: 17613 - RNA, 20 nt, synthetic construct
  source 1..20: mol_type = other RNA
tctcttattacatgaagaca

SEQ ID NO: 17614 - RNA, 20 nt, synthetic construct
  source 1..20: mol_type = other RNA
tgggtgaaaattagttctta

SEQ ID NO: 17615 - RNA, 20 nt, synthetic construct
  source 1..20: mol_type = other RNA
actcaggctggagtgtgcag

SEQ ID NO: 17616 - RNA, 20 nt, synthetic construct
  source 1..20: mol_type = other RNA
tctcactctatcactcaggc

SEQ ID NO: 17617 - RNA, 20 nt, synthetic construct
  source 1..20: mol_type = other RNA
agagtctcactctatcactc

SEQ ID NO: 17618 - RNA, 20 nt, synthetic construct
  source 1..20: mol_type = other RNA
aaaaaactattaattgatat

SEQ ID NO: 17619 - RNA, 20 nt, synthetic construct
  source 1..20: mol_type = other RNA
gttttttactaacttagata

SEQ ID NO: 17620 - RNA, 20 nt, synthetic construct
  source 1..20: mol_type = other RNA
ccacaaaaattatgaaactg

SEQ ID NO: 17621 - RNA, 20 nt, synthetic construct
  source 1..20: mol_type = other RNA
cctcagtttcataatttttg

SEQ ID NO: 17622 - RNA, 20 nt, synthetic construct
  source 1..20: mol_type = other RNA
actgaggaaaatacttgaaa

SEQ ID NO: 17623 - RNA, 20 nt, synthetic construct
  source 1..20: mol_type = other RNA
gaggaaaatacttgaaaagg

SEQ ID NO: 17624 - RNA, 20 nt, synthetic construct
  source 1..20: mol_type = other RNA
gaaaatacttgaaaaggtgg

SEQ ID NO: 17625 - RNA, 20 nt, synthetic construct
  source 1..20: mol_type = other RNA
gaaaaggtggaggctgcatc

SEQ ID NO: 17626 - RNA, 20 nt, synthetic construct
  source 1..20: mol_type = other RNA
ggatttacctctgaagaaaa

SEQ ID NO: 17627 - RNA, 20 nt, synthetic construct
  source 1..20: mol_type = other RNA
atggtcacctttttcttcag

SEQ ID NO: 17628 - RNA, 20 nt, synthetic construct
  source 1..20: mol_type = other RNA
ttaacgcatataagttaaga

SEQ ID NO: 17629 - RNA, 20 nt, synthetic construct
  source 1..20: mol_type = other RNA
gaaatgtgtgtctgtgtagt

SEQ ID NO: 17630 - RNA, 20 nt, synthetic construct
  source 1..20: mol_type = other RNA
aaatgtgtgtctgtgtagtt

SEQ ID NO: 17631 - RNA, 20 nt, synthetic construct
  source 1..20: mol_type = other RNA
aatgtgtgtctgtgtagttg

SEQ ID NO: 17632 - RNA, 20 nt, synthetic construct
  source 1..20: mol_type = other RNA
atgtgtgtctgtgtagttgg

SEQ ID NO: 17633 - RNA, 20 nt, synthetic construct
  source 1..20: mol_type = other RNA
tgtgtgtctgtgtagttggg

SEQ ID NO: 17634 - RNA, 20 nt, synthetic construct
  source 1..20: mol_type = other RNA
ttaaaaatcaaataagtcac

SEQ ID NO: 17635 - RNA, 20 nt, synthetic construct
  source 1..20: mol_type = other RNA
aaattttctcctagatcctg

SEQ ID NO: 17636 - RNA, 20 nt, synthetic construct
  source 1..20: mol_type = other RNA
tcaagaattcctcaggatct

SEQ ID NO: 17637 - RNA, 20 nt, synthetic construct
  source 1..20: mol_type = other RNA
agaatattcaagaattcctc

SEQ ID NO: 17638 - RNA, 20 nt, synthetic construct
  source 1..20: mol_type = other RNA
ttctgtttcatcatatttta

SEQ ID NO: 17639 - RNA, 20 nt, synthetic construct
  source 1..20: mol_type = other RNA
tctgtttcatcatattttaa

SEQ ID NO: 17640 - RNA, 20 nt, synthetic construct
  source 1..20: mol_type = other RNA
tagaacctttgctaaaaata

SEQ ID NO: 17641 - RNA, 20 nt, synthetic construct
  source 1..20: mol_type = other RNA
ggttaccttatttttagcaa

SEQ ID NO: 17642 - RNA, 20 nt, synthetic construct
  source 1..20: mol_type = other RNA
ttaaattgttctagaagcat

SEQ ID NO: 17643 - RNA, 20 nt, synthetic construct
  source 1..20: mol_type = other RNA
atgcttctagaacaatttaa

SEQ ID NO: 17644 - RNA, 20 nt, synthetic construct
  source 1..20: mol_type = other RNA
aaatcatgtctgttgaataa

SEQ ID NO: 17645 - RNA, 20 nt, synthetic construct
  source 1..20: mol_type = other RNA
acaatattaagaaatcattc

SEQ ID NO: 17646 - RNA, 20 nt, synthetic construct
  source 1..20: mol_type = other RNA
tcttaatattgtatttgttt

SEQ ID NO: 17647 - RNA, 20 nt, synthetic construct
  source 1..20: mol_type = other RNA
cttaatattgtatttgttta

SEQ ID NO: 17648 - RNA, 20 nt, synthetic construct
  source 1..20: mol_type = other RNA
atttgtttagggctcttaat

SEQ ID NO: 17649 - RNA, 20 nt, synthetic construct
  source 1..20: mol_type = other RNA
aagctacaccatcaatttta

SEQ ID NO: 17650 - RNA, 20 nt, synthetic construct
  source 1..20: mol_type = other RNA
taaaattgatggtgtagctt

SEQ ID NO: 17651 - RNA, 20 nt, synthetic construct
  source 1..20: mol_type = other RNA
cagaaaaaccataaaattga

SEQ ID NO: 17652 - RNA, 20 nt, synthetic construct
  source 1..20: mol_type = other RNA
tttctgttctcaaatactgc

SEQ ID NO: 17653 - RNA, 20 nt, synthetic construct
  source 1..20: mol_type = other RNA
ttctgttctcaaatactgct

SEQ ID NO: 17654 - RNA, 20 nt, synthetic construct
  source 1..20: mol_type = other RNA
gatttaagcatttgataaat

SEQ ID NO: 17655 - RNA, 20 nt, synthetic construct
  source 1..20: mol_type = other RNA
ctgcgtgtttttagatcagc

SEQ ID NO: 17656 - RNA, 20 nt, synthetic construct
  source 1..20: mol_type = other RNA
ttttagatcagcaggtcaaa

SEQ ID NO: 17657 - RNA, 20 nt, synthetic construct
  source 1..20: mol_type = other RNA
ttacttctatcaaattttta

SEQ ID NO: 17658 - RNA, 20 nt, synthetic construct
  source 1..20: mol_type = other RNA
atggaaaaaaatgagaaagt

SEQ ID NO: 17659 - RNA, 20 nt, synthetic construct
  source 1..20: mol_type = other RNA
caattcagcagttgttagaa

SEQ ID NO: 17660 - RNA, 20 nt, synthetic construct
  source 1..20: mol_type = other RNA
tctaacaactgctgaattgt

SEQ ID NO: 17661 - RNA, 20 nt, synthetic construct
  source 1..20: mol_type = other RNA
ttctaacaactgctgaattg

SEQ ID NO: 17662 - RNA, 20 nt, synthetic construct
  source 1..20: mol_type = other RNA
cagtaacctgaaatttgcag

SEQ ID NO: 17663 - RNA, 20 nt, synthetic construct
  source 1..20: mol_type = other RNA
cactaacctctgcaaatttc

SEQ ID NO: 17664 - RNA, 20 nt, synthetic construct
  source 1..20: mol_type = other RNA
aggttagtgatactcacctg

SEQ ID NO: 17665 - RNA, 20 nt, synthetic construct
  source 1..20: mol_type = other RNA
actttcacataaaataccac

SEQ ID NO: 17666 - RNA, 20 nt, synthetic construct
  source 1..20: mol_type = other RNA
gtattttatgtgaaagtctg

SEQ ID NO: 17667 - RNA, 20 nt, synthetic construct
  source 1..20: mol_type = other RNA
tattttatgtgaaagtctgt

SEQ ID NO: 17668 - RNA, 20 nt, synthetic construct
  source 1..20: mol_type = other RNA
tgtgggagtcttaagactat

SEQ ID NO: 17669 - RNA, 20 nt, synthetic construct
  source 1..20: mol_type = other RNA
ttcataggacaccaatatta

SEQ ID NO: 17670 - RNA, 20 nt, synthetic construct
  source 1..20: mol_type = other RNA
aaacagttctgccttaatat

SEQ ID NO: 17671 - RNA, 20 nt, synthetic construct
  source 1..20: mol_type = other RNA
tttgacagccatgactattt

SEQ ID NO: 17672 - RNA, 20 nt, synthetic construct
  source 1..20: mol_type = other RNA
catgactattttggtttcat

SEQ ID NO: 17673 - RNA, 20 nt, synthetic construct
  source 1..20: mol_type = other RNA
atgactattttggtttcata

SEQ ID NO: 17674 - RNA, 20 nt, synthetic construct
  source 1..20: mol_type = other RNA
ctatgaaaccaaaatagtca

SEQ ID NO: 17675 - RNA, 20 nt, synthetic construct
  source 1..20: mol_type = other RNA
aaaatatctgtcttttttat

SEQ ID NO: 17676 - RNA, 20 nt, synthetic construct
  source 1..20: mol_type = other RNA
atctgaataatcagacatga

SEQ ID NO: 17677 - RNA, 20 nt, synthetic construct
  source 1..20: mol_type = other RNA
attattcagatgcctcgatt

SEQ ID NO: 17678 - RNA, 20 nt, synthetic construct
  source 1..20: mol_type = other RNA
ttaaagtcttttccaaatcg

SEQ ID NO: 17679 - RNA, 20 nt, synthetic construct
  source 1..20: mol_type = other RNA
taaaaaaatttttccttctc

SEQ ID NO: 17680 - RNA, 20 nt, synthetic construct
  source 1..20: mol_type = other RNA
gttatatttaattccagaga

SEQ ID NO: 17681 - RNA, 20 nt, synthetic construct
  source 1..20: mol_type = other RNA
atttttttagtttgttttgt

SEQ ID NO: 17682 - RNA, 20 nt, synthetic construct
  source 1..20: mol_type = other RNA
agtttgttttgttggttttg

SEQ ID NO: 17683 - RNA, 20 nt, synthetic construct
  source 1..20: mol_type = other RNA
cagataattctcatcagttg

SEQ ID NO: 17684 - RNA, 20 nt, synthetic construct
  source 1..20: mol_type = other RNA
agataattctcatcagttgt

SEQ ID NO: 17685 - RNA, 20 nt, synthetic construct
  source 1..20: mol_type = other RNA
gttgtgggttagactctaac

SEQ ID NO: 17686 - RNA, 20 nt, synthetic construct
  source 1..20: mol_type = other RNA
actggacacagtatttccca

SEQ ID NO: 17687 - RNA, 20 nt, synthetic construct
  source 1..20: mol_type = other RNA
ttcagatactgaattgcctt

SEQ ID NO: 17688 - RNA, 20 nt, synthetic construct
  source 1..20: mol_type = other RNA
tttaaaaaggacaatgttca

SEQ ID NO: 17689 - RNA, 20 nt, synthetic construct
  source 1..20: mol_type = other RNA
agaaaagttaggctttaaaa

SEQ ID NO: 17690 - RNA, 20 nt, synthetic construct
  source 1..20: mol_type = other RNA
agaagatgtaaagaaaagtt

SEQ ID NO: 17691 - RNA, 20 nt, synthetic construct
  source 1..20: mol_type = other RNA
gaaggggaagggaagttaag

SEQ ID NO: 17692 - RNA, 20 nt, synthetic construct
  source 1..20: mol_type = other RNA
ctgaaatgtgagaaggggaa

SEQ ID NO: 17693 - RNA, 20 nt, synthetic construct
  source 1..20: mol_type = other RNA
gctgaaatgtgagaagggga

SEQ ID NO: 17694 - RNA, 20 nt, synthetic construct
  source 1..20: mol_type = other RNA
gggagctgaaatgtgagaag

SEQ ID NO: 17695 - RNA, 20 nt, synthetic construct
  source 1..20: mol_type = other RNA
tgggagctgaaatgtgagaa

SEQ ID NO: 17696 - RNA, 20 nt, synthetic construct
  source 1..20: mol_type = other RNA
ctgggagctgaaatgtgaga

SEQ ID NO: 17697 - RNA, 20 nt, synthetic construct
  source 1..20: mol_type = other RNA
tttcagctcccagacagtgc

SEQ ID NO: 17698 - RNA, 20 nt, synthetic construct
  source 1..20: mol_type = other RNA
cccagacagtgccggatatg

SEQ ID NO: 17699 - RNA, 20 nt, synthetic construct
  source 1..20: mol_type = other RNA
agacagtgccggatatgtgg

SEQ ID NO: 17700 - RNA, 20 nt, synthetic construct
  source 1..20: mol_type = other RNA
gacagtgccggatatgtgga

SEQ ID NO: 17701 - RNA, 20 nt, synthetic construct
  source 1..20: mol_type = other RNA
ccacatatccggcactgtct

SEQ ID NO: 17702 - RNA, 20 nt, synthetic construct
  source 1..20: mol_type = other RNA
tccacatatccggcactgtc

SEQ ID NO: 17703 - RNA, 20 nt, synthetic construct
  source 1..20: mol_type = other RNA
ttgcaagccctccacatatc

SEQ ID NO: 17704 - RNA, 20 nt, synthetic construct
  source 1..20: mol_type = other RNA
tagagaatgctacgacgatc

SEQ ID NO: 17705 - RNA, 20 nt, synthetic construct
  source 1..20: mol_type = other RNA
gacgatccggacatctcagc

SEQ ID NO: 17706 - RNA, 20 nt, synthetic construct
  source 1..20: mol_type = other RNA
atttttccagctgagatgtc

SEQ ID NO: 17707 - RNA, 20 nt, synthetic construct
  source 1..20: mol_type = other RNA
gaagctcacttgagtgttgc

SEQ ID NO: 17708 - RNA, 20 nt, synthetic construct
  source 1..20: mol_type = other RNA
gtgagcttcccttcacttaa

SEQ ID NO: 17709 - RNA, 20 nt, synthetic construct
  source 1..20: mol_type = other RNA
aagtttatccattaagtgaa

SEQ ID NO: 17710 - RNA, 20 nt, synthetic construct
  source 1..20: mol_type = other RNA
aaagtttatccattaagtga

SEQ ID NO: 17711 - RNA, 20 nt, synthetic construct
  source 1..20: mol_type = other RNA
tgaaaacacaatgctcgttt

SEQ ID NO: 17712 - RNA, 20 nt, synthetic construct
  source 1..20: mol_type = other RNA
ttttttaaaatcataattaa

SEQ ID NO: 17713 - RNA, 20 nt, synthetic construct
  source 1..20: mol_type = other RNA
taaaaatacaaaaattagct

SEQ ID NO: 17714 - RNA, 20 nt, synthetic construct
  source 1..20: mol_type = other RNA
ttaaaaatacaaaaattagc

SEQ ID NO: 17715 - RNA, 20 nt, synthetic construct
  source 1..20: mol_type = other RNA
tttgtatttttaacagagac

SEQ ID NO: 17716 - RNA, 20 nt, synthetic construct
  source 1..20: mol_type = other RNA
ttgtatttttaacagagaca

SEQ ID NO: 17717 - RNA, 20 nt, synthetic construct
  source 1..20: mol_type = other RNA
agggtttcaccatcttgatc

SEQ ID NO: 17718 - RNA, 20 nt, synthetic construct
  source 1..20: mol_type = other RNA
tttcaccatcttgatcaggc

SEQ ID NO: 17719 - RNA, 20 nt, synthetic construct
  source 1..20: mol_type = other RNA
caagaccagcctgatcaaga

SEQ ID NO: 17720 - RNA, 20 nt, synthetic construct
  source 1..20: mol_type = other RNA
acctcgtgatccaccagcct

SEQ ID NO: 17721 - RNA, 20 nt, synthetic construct
  source 1..20: mol_type = other RNA
ggctggtggatcacgaggtc

SEQ ID NO: 17722 - RNA, 20 nt, synthetic construct
  source 1..20: mol_type = other RNA
gccgaggctggtggatcacg

SEQ ID NO: 17723 - RNA, 20 nt, synthetic construct
  source 1..20: mol_type = other RNA
tgtcattaggccgaggctgg

SEQ ID NO: 17724 - RNA, 20 nt, synthetic construct
  source 1..20: mol_type = other RNA
gaatgtcattaggccgaggc

SEQ ID NO: 17725 - RNA, 20 nt, synthetic construct
  source 1..20: mol_type = other RNA
gcctaatgacattcttttca

SEQ ID NO: 17726 - RNA, 20 nt, synthetic construct
  source 1..20: mol_type = other RNA
accatgaaaagaatgtcatt

SEQ ID NO: 17727 - RNA, 20 nt, synthetic construct
  source 1..20: mol_type = other RNA
ttcttttcatggtccatttt

SEQ ID NO: 17728 - RNA, 20 nt, synthetic construct
  source 1..20: mol_type = other RNA
ggatgaaggtggacctaaaa

SEQ ID NO: 17729 - RNA, 20 nt, synthetic construct
  source 1..20: mol_type = other RNA
aggtccaccttcatccgaag

SEQ ID NO: 17730 - RNA, 20 nt, synthetic construct
  source 1..20: mol_type = other RNA
tcagcctcttcggatgaagg

SEQ ID NO: 17731 - RNA, 20 nt, synthetic construct
  source 1..20: mol_type = other RNA
gattcagcctcttcggatga

SEQ ID NO: 17732 - RNA, 20 nt, synthetic construct
  source 1..20: mol_type = other RNA
tatttatgattcagcctctt

SEQ ID NO: 17733 - RNA, 20 nt, synthetic construct
  source 1..20: mol_type = other RNA
agtctttgggaagtgacact

SEQ ID NO: 17734 - RNA, 20 nt, synthetic construct
  source 1..20: mol_type = other RNA
aagtctttgggaagtgacac

SEQ ID NO: 17735 - RNA, 20 nt, synthetic construct
  source 1..20: mol_type = other RNA
ttcccaaagacttacccgac

SEQ ID NO: 17736 - RNA, 20 nt, synthetic construct
  source 1..20: mol_type = other RNA
tcccaaagacttacccgact

SEQ ID NO: 17737 - RNA, 20 nt, synthetic construct
  source 1..20: mol_type = other RNA
aagacttacccgactgggac

SEQ ID NO: 17738 - RNA, 20 nt, synthetic construct
  source 1..20: mol_type = other RNA
tcccagtcgggtaagtcttt

SEQ ID NO: 17739 - RNA, 20 nt, synthetic construct
  source 1..20: mol_type = other RNA
gtcccagtcgggtaagtctt

SEQ ID NO: 17740 - RNA, 20 nt, synthetic construct
  source 1..20: mol_type = other RNA
cccgactgggactggagaca

SEQ ID NO: 17741 - RNA, 20 nt, synthetic construct
  source 1..20: mol_type = other RNA
ccgtgtctccagtcccagtc

SEQ ID NO: 17742 - RNA, 20 nt, synthetic construct
  source 1..20: mol_type = other RNA
gccgtgtctccagtcccagt

SEQ ID NO: 17743 - RNA, 20 nt, synthetic construct
  source 1..20: mol_type = other RNA
ctgcatcccttgccagaata

SEQ ID NO: 17744 - RNA, 20 nt, synthetic construct
  source 1..20: mol_type = other RNA
ataactccatattctggcaa

SEQ ID NO: 17745 - RNA, 20 nt, synthetic construct
  source 1..20: mol_type = other RNA
aataactccatattctggca

SEQ ID NO: 17746 - RNA, 20 nt, synthetic construct
  source 1..20: mol_type = other RNA
cagcaaataactccatattc

SEQ ID NO: 17747 - RNA, 20 nt, synthetic construct
  source 1..20: mol_type = other RNA
tatgttgcttttgtgaagta

SEQ ID NO: 17748 - RNA, 20 nt, synthetic construct
  source 1..20: mol_type = other RNA
acttcacaaaagcaacatag

SEQ ID NO: 17749 - RNA, 20 nt, synthetic construct
  source 1..20: mol_type = other RNA
tgcttttgtgaagtatggga

SEQ ID NO: 17750 - RNA, 20 nt, synthetic construct
  source 1..20: mol_type = other RNA
atgggaaggacgattctgcc

SEQ ID NO: 17751 - RNA, 20 nt, synthetic construct
  source 1..20: mol_type = other RNA
ctggctcttctttgacagca

SEQ ID NO: 17752 - RNA, 20 nt, synthetic construct
  source 1..20: mol_type = other RNA
catgctgtcaaagaagagcc

SEQ ID NO: 17753 - RNA, 20 nt, synthetic construct
  source 1..20: mol_type = other RNA
tctttgacagcatggccgat

SEQ ID NO: 17754 - RNA, 20 nt, synthetic construct
  source 1..20: mol_type = other RNA
ctttgacagcatggccgatc

SEQ ID NO: 17755 - RNA, 20 nt, synthetic construct
  source 1..20: mol_type = other RNA
gacagcatggccgatcggga

SEQ ID NO: 17756 - RNA, 20 nt, synthetic construct
  source 1..20: mol_type = other RNA
gttttcagtaccatcccgat

SEQ ID NO: 17757 - RNA, 20 nt, synthetic construct
  source 1..20: mol_type = other RNA
aaacgcctttcttctgcatg

SEQ ID NO: 17758 - RNA, 20 nt, synthetic construct
  source 1..20: mol_type = other RNA
ctttcttctgcatgtggcac

SEQ ID NO: 17759 - RNA, 20 nt, synthetic construct
  source 1..20: mol_type = other RNA
tttcttctgcatgtggcaca

SEQ ID NO: 17760 - RNA, 20 nt, synthetic construct
  source 1..20: mol_type = other RNA
ctgtgccacatgcagaagaa

SEQ ID NO: 17761 - RNA, 20 nt, synthetic construct
  source 1..20: mol_type = other RNA
ctgcatgtggcacagggttc

SEQ ID NO: 17762 - RNA, 20 nt, synthetic construct
  source 1..20: mol_type = other RNA
cacagggttctggtttgtag

SEQ ID NO: 17763 - RNA, 20 nt, synthetic construct
  source 1..20: mol_type = other RNA
acagggttctggtttgtagt

SEQ ID NO: 17764 - RNA, 20 nt, synthetic construct
  source 1..20: mol_type = other RNA
tgtagtgggacagtttgtag

SEQ ID NO: 17765 - RNA, 20 nt, synthetic construct
  source 1..20: mol_type = other RNA
gtagtgggacagtttgtagt

SEQ ID NO: 17766 - RNA, 20 nt, synthetic construct
  source 1..20: mol_type = other RNA
cagaaaatatcactcagaac

SEQ ID NO: 17767 - RNA, 20 nt, synthetic construct
  source 1..20: mol_type = other RNA
ttttctgagaaaatcctttc

SEQ ID NO: 17768 - RNA, 20 nt, synthetic construct
  source 1..20: mol_type = other RNA
aaatcctttcaggattattc

SEQ ID NO: 17769 - RNA, 20 nt, synthetic construct
  source 1..20: mol_type = other RNA
agagcctgaaattagctttt

SEQ ID NO: 17770 - RNA, 20 nt, synthetic construct
  source 1..20: mol_type = other RNA
atttccaaaaagctaatttc

SEQ ID NO: 17771 - RNA, 20 nt, synthetic construct
  source 1..20: mol_type = other RNA
attagctttttggaaatgat

SEQ ID NO: 17772 - RNA, 20 nt, synthetic construct
  source 1..20: mol_type = other RNA
tgataggattataaaatcac

SEQ ID NO: 17773 - RNA, 20 nt, synthetic construct
  source 1..20: mol_type = other RNA
attataaaatcactggcaaa

SEQ ID NO: 17774 - RNA, 20 nt, synthetic construct
  source 1..20: mol_type = other RNA
ttataaaatcactggcaaaa

SEQ ID NO: 17775 - RNA, 20 nt, synthetic construct
  source 1..20: mol_type = other RNA
cagaggaagaactctttata

SEQ ID NO: 17776 - RNA, 20 nt, synthetic construct
  source 1..20: mol_type = other RNA
acagaggaagaactctttat

SEQ ID NO: 17777 - RNA, 20 nt, synthetic construct
  source 1..20: mol_type = other RNA
gagttcttcctctgtgccat

SEQ ID NO: 17778 - RNA, 20 nt, synthetic construct
  source 1..20: mol_type = other RNA
ttcttcctctgtgccatagg

SEQ ID NO: 17779 - RNA, 20 nt, synthetic construct
  source 1..20: mol_type = other RNA
tgtgccataggtggtcagaa

SEQ ID NO: 17780 - RNA, 20 nt, synthetic construct
  source 1..20: mol_type = other RNA
tctgaccacctatggcacag

SEQ ID NO: 17781 - RNA, 20 nt, synthetic construct
  source 1..20: mol_type = other RNA
gaagccattctgaccaccta

SEQ ID NO: 17782 - RNA, 20 nt, synthetic construct
  source 1..20: mol_type = other RNA
tctgggcatggggtgacttg

SEQ ID NO: 17783 - RNA, 20 nt, synthetic construct
  source 1..20: mol_type = other RNA
gtcaccccatgcccagaagt

SEQ ID NO: 17784 - RNA, 20 nt, synthetic construct
  source 1..20: mol_type = other RNA
ctctcctacttctgggcatg

SEQ ID NO: 17785 - RNA, 20 nt, synthetic construct
  source 1..20: mol_type = other RNA
actctcctacttctgggcat

SEQ ID NO: 17786 - RNA, 20 nt, synthetic construct
  source 1..20: mol_type = other RNA
tactctcctacttctgggca

SEQ ID NO: 17787 - RNA, 20 nt, synthetic construct
  source 1..20: mol_type = other RNA
tcaagtactctcctacttct

SEQ ID NO: 17788 - RNA, 20 nt, synthetic construct
  source 1..20: mol_type = other RNA
ttcaagtactctcctacttc

SEQ ID NO: 17789 - RNA, 20 nt, synthetic construct
  source 1..20: mol_type = other RNA
agagtacttgaagatgtctc

SEQ ID NO: 17790 - RNA, 20 nt, synthetic construct
  source 1..20: mol_type = other RNA
tctggaagacctgcattcct

SEQ ID NO: 17791 - RNA, 20 nt, synthetic construct
  source 1..20: mol_type = other RNA
acctgcattccttggactcc

SEQ ID NO: 17792 - RNA, 20 nt, synthetic construct
  source 1..20: mol_type = other RNA
tcctggagtccaaggaatgc

SEQ ID NO: 17793 - RNA, 20 nt, synthetic construct
  source 1..20: mol_type = other RNA
ttggactccaggagaatcca

SEQ ID NO: 17794 - RNA, 20 nt, synthetic construct
  source 1..20: mol_type = other RNA
ttggattctcctggagtcca

SEQ ID NO: 17795 - RNA, 20 nt, synthetic construct
  source 1..20: mol_type = other RNA
tgcacagccttggattctcc

SEQ ID NO: 17796 - RNA, 20 nt, synthetic construct
  source 1..20: mol_type = other RNA
gcagtcttcgtgcacagcct

SEQ ID NO: 17797 - RNA, 20 nt, synthetic construct
  source 1..20: mol_type = other RNA
acaaactcattgttggactc

SEQ ID NO: 17798 - RNA, 20 nt, synthetic construct
  source 1..20: mol_type = other RNA
aatgagtttgtacaaataac

SEQ ID NO: 17799 - RNA, 20 nt, synthetic construct
  source 1..20: mol_type = other RNA
atgagtttgtacaaataact

SEQ ID NO: 17800 - RNA, 20 nt, synthetic construct
  source 1..20: mol_type = other RNA
tgagtttgtacaaataactg

SEQ ID NO: 17801 - RNA, 20 nt, synthetic construct
  source 1..20: mol_type = other RNA
gtacaaataactggggtcat

SEQ ID NO: 17802 - RNA, 20 nt, synthetic construct
  source 1..20: mol_type = other RNA
tacaaataactggggtcatc

SEQ ID NO: 17803 - RNA, 20 nt, synthetic construct
  source 1..20: mol_type = other RNA
ataactggggtcatcgggaa

SEQ ID NO: 17804 - RNA, 20 nt, synthetic construct
  source 1..20: mol_type = other RNA
gggaaaggcaaagaaactga

SEQ ID NO: 17805 - RNA, 20 nt, synthetic construct
  source 1..20: mol_type = other RNA
acgttgcatcttattcgagc

SEQ ID NO: 17806 - RNA, 20 nt, synthetic construct
  source 1..20: mol_type = other RNA
ctcgaataagatgcaacgtt

SEQ ID NO: 17807 - RNA, 20 nt, synthetic construct
  source 1..20: mol_type = other RNA
gttctgttcacgtccattgc

SEQ ID NO: 17808 - RNA, 20 nt, synthetic construct
  source 1..20: mol_type = other RNA
ttcacgtccattgccggcaa

SEQ ID NO: 17809 - RNA, 20 nt, synthetic construct
  source 1..20: mol_type = other RNA
aagacatccattgccggcaa

SEQ ID NO: 17810 - RNA, 20 nt, synthetic construct
  source 1..20: mol_type = other RNA
accacaaagacatccattgc

SEQ ID NO: 17811 - RNA, 20 nt, synthetic construct
  source 1..20: mol_type = other RNA
tggtgatgatccttcagaaa

SEQ ID NO: 17812 - RNA, 20 nt, synthetic construct
  source 1..20: mol_type = other RNA
acagaggcatccttttctga

SEQ ID NO: 17813 - RNA, 20 nt, synthetic construct
  source 1..20: mol_type = other RNA
agcaatttgtttttaaacag

SEQ ID NO: 17814 - RNA, 20 nt, synthetic construct
  source 1..20: mol_type = other RNA
gcttcttattaaatacttca

SEQ ID NO: 17815 - RNA, 20 nt, synthetic construct
  source 1..20: mol_type = other RNA
tgcttcttattaaatacttc

SEQ ID NO: 17816 - RNA, 20 nt, synthetic construct
  source 1..20: mol_type = other RNA
tctagaaagtatgtttgtgt

SEQ ID NO: 17817 - RNA, 20 nt, synthetic construct
  source 1..20: mol_type = other RNA
tgcacttaacttaaagcttc

SEQ ID NO: 17818 - RNA, 20 nt, synthetic construct
  source 1..20: mol_type = other RNA
cattgatcatatgatatttt

SEQ ID NO: 17819 - RNA, 20 nt, synthetic construct
  source 1..20: mol_type = other RNA
gaagcatacaattttaattg

SEQ ID NO: 17820 - RNA, 20 nt, synthetic construct
  source 1..20: mol_type = other RNA
cattctcaatggactaaaag

SEQ ID NO: 17821 - RNA, 20 nt, synthetic construct
  source 1..20: mol_type = other RNA
acatttatttacattctcaa

SEQ ID NO: 17822 - RNA, 20 nt, synthetic construct
  source 1..20: mol_type = other RNA
aaataaatgtgtcttcttta

SEQ ID NO: 17823 - RNA, 20 nt, synthetic construct
  source 1..20: mol_type = other RNA
tgtgtcttctttatggacca

SEQ ID NO: 17824 - RNA, 20 nt, synthetic construct
  source 1..20: mol_type = other RNA
gaaaaatgatttcatatcct

SEQ ID NO: 17825 - RNA, 20 nt, synthetic construct
  source 1..20: mol_type = other RNA
catttttcttttgtagctaa

SEQ ID NO: 17826 - RNA, 20 nt, synthetic construct
  source 1..20: mol_type = other RNA
tgtagctaacggttgccttg

SEQ ID NO: 17827 - RNA, 20 nt, synthetic construct
  source 1..20: mol_type = other RNA
gccttgaggaagaaataatt

SEQ ID NO: 17828 - RNA, 20 nt, synthetic construct
  source 1..20: mol_type = other RNA
accaaattatttcttcctca

SEQ ID NO: 17829 - RNA, 20 nt, synthetic construct
  source 1..20: mol_type = other RNA
ctcagtacatctctaataac

SEQ ID NO: 17830 - RNA, 20 nt, synthetic construct
  source 1..20: mol_type = other RNA
aagatcagcagtatatagaa

SEQ ID NO: 17831 - RNA, 20 nt, synthetic construct
  source 1..20: mol_type = other RNA
tttctgtgtttctgcaatag

SEQ ID NO: 17832 - RNA, 20 nt, synthetic construct
  source 1..20: mol_type = other RNA
aaatacttaaattcccttaa

SEQ ID NO: 17833 - RNA, 20 nt, synthetic construct
  source 1..20: mol_type = other RNA
atagaaaacaacaccattaa

SEQ ID NO: 17834 - RNA, 20 nt, synthetic construct
  source 1..20: mol_type = other RNA
aatagaaaacaacaccatta

SEQ ID NO: 17835 - RNA, 20 nt, synthetic construct
  source 1..20: mol_type = other RNA
gtgttgttttctatttgttc

SEQ ID NO: 17836 - RNA, 20 nt, synthetic construct
  source 1..20: mol_type = other RNA
acttcaaaaatggacatttg

SEQ ID NO: 17837 - RNA, 20 nt, synthetic construct
  source 1..20: mol_type = other RNA
cacttcaaaaatggacattt

SEQ ID NO: 17838 - RNA, 20 nt, synthetic construct
  source 1..20: mol_type = other RNA
tcacttcaaaaatggacatt

SEQ ID NO: 17839 - RNA, 20 nt, synthetic construct
  source 1..20: mol_type = other RNA
catttttgaagtgattttcc

SEQ ID NO: 17840 - RNA, 20 nt, synthetic construct
  source 1..20: mol_type = other RNA
ttttgaagtgattttcctgg

SEQ ID NO: 17841 - RNA, 20 nt, synthetic construct
  source 1..20: mol_type = other RNA
caggaaaatcacttcaaaaa

SEQ ID NO: 17842 - RNA, 20 nt, synthetic construct
  source 1..20: mol_type = other RNA
agtgattttcctggaggatt

SEQ ID NO: 17843 - RNA, 20 nt, synthetic construct
  source 1..20: mol_type = other RNA
gtgattttcctggaggatta

SEQ ID NO: 17844 - RNA, 20 nt, synthetic construct
  source 1..20: mol_type = other RNA
gctaaataccctaatcctcc

SEQ ID NO: 17845 - RNA, 20 nt, synthetic construct
  source 1..20: mol_type = other RNA
agtagttactgtcagctaac

SEQ ID NO: 17846 - RNA, 20 nt, synthetic construct
  source 1..20: mol_type = other RNA
gtcagctaacaggtttttta

SEQ ID NO: 17847 - RNA, 20 nt, synthetic construct
  source 1..20: mol_type = other RNA
ttttaactattaatatttta

SEQ ID NO: 17848 - RNA, 20 nt, synthetic construct
  source 1..20: mol_type = other RNA
actattaatattttatggaa

SEQ ID NO: 17849 - RNA, 20 nt, synthetic construct
  source 1..20: mol_type = other RNA
ctattaatattttatggaat

SEQ ID NO: 17850 - RNA, 20 nt, synthetic construct
  source 1..20: mol_type = other RNA
tattaatattttatggaatg

SEQ ID NO: 17851 - RNA, 20 nt, synthetic construct
  source 1..20: mol_type = other RNA
aagtaaattgatgaaagaat

SEQ ID NO: 17852 - RNA, 20 nt, synthetic construct
  source 1..20: mol_type = other RNA
tatggactgtatgtttgtaa

SEQ ID NO: 17853 - RNA, 20 nt, synthetic construct
  source 1..20: mol_type = other RNA
agtccataagaaaatgaatt

SEQ ID NO: 17854 - RNA, 20 nt, synthetic construct
  source 1..20: mol_type = other RNA
atgccaaattcattttctta

SEQ ID NO: 17855 - RNA, 20 nt, synthetic construct
  source 1..20: mol_type = other RNA
atagaattattacaatttcc

SEQ ID NO: 17856 - RNA, 20 nt, synthetic construct
  source 1..20: mol_type = other RNA
tagaattattacaatttcct

SEQ ID NO: 17857 - RNA, 20 nt, synthetic construct
  source 1..20: mol_type = other RNA
ttacaatttcctgggagaga

SEQ ID NO: 17858 - RNA, 20 nt, synthetic construct
  source 1..20: mol_type = other RNA
tttaaatatccatctctccc

SEQ ID NO: 17859 - RNA, 20 nt, synthetic construct
  source 1..20: mol_type = other RNA
agtcttgtctaaaataatag

SEQ ID NO: 17860 - RNA, 20 nt, synthetic construct
  source 1..20: mol_type = other RNA
actgaatttaatgggagtac

SEQ ID NO: 17861 - RNA, 20 nt, synthetic construct
  source 1..20: mol_type = other RNA
gaaactacactgaatttaat

SEQ ID NO: 17862 - RNA, 20 nt, synthetic construct
  source 1..20: mol_type = other RNA
tgaaactacactgaatttaa

SEQ ID NO: 17863 - RNA, 20 nt, synthetic construct
  source 1..20: mol_type = other RNA
tacttactttaatcagaagg

SEQ ID NO: 17864 - RNA, 20 nt, synthetic construct
  source 1..20: mol_type = other RNA
ctgattaaagtaagtagaaa

SEQ ID NO: 17865 - RNA, 20 nt, synthetic construct
  source 1..20: mol_type = other RNA
ttctacttactttaatcaga

SEQ ID NO: 17866 - RNA, 20 nt, synthetic construct
  source 1..20: mol_type = other RNA
agtgtgtgtttagaccacag

SEQ ID NO: 17867 - RNA, 20 nt, synthetic construct
  source 1..20: mol_type = other RNA
tgtggtctaaacacacacta

SEQ ID NO: 17868 - RNA, 20 nt, synthetic construct
  source 1..20: mol_type = other RNA
cacagcggatgttgtagacc

SEQ ID NO: 17869 - RNA, 20 nt, synthetic construct
  source 1..20: mol_type = other RNA
ctggtctacaacatccgctg

SEQ ID NO: 17870 - RNA, 20 nt, synthetic construct
  source 1..20: mol_type = other RNA
acatgtatcatctatggtcc

SEQ ID NO: 17871 - RNA, 20 nt, synthetic construct
  source 1..20: mol_type = other RNA
gcactgacatgtatcatcta

SEQ ID NO: 17872 - RNA, 20 nt, synthetic construct
  source 1..20: mol_type = other RNA
attctctgagtgttgttttg

SEQ ID NO: 17873 - RNA, 20 nt, synthetic construct
  source 1..20: mol_type = other RNA
gcacagttagaaagtcattc

SEQ ID NO: 17874 - RNA, 20 nt, synthetic construct
  source 1..20: mol_type = other RNA
gactttctaactgtgcagaa

SEQ ID NO: 17875 - RNA, 20 nt, synthetic construct
  source 1..20: mol_type = other RNA
atatttaatgtgacaaaaag

SEQ ID NO: 17876 - RNA, 20 nt, synthetic construct
  source 1..20: mol_type = other RNA
ccctgcaattacttttttaa

SEQ ID NO: 17877 - RNA, 20 nt, synthetic construct
  source 1..20: mol_type = other RNA
cctttaaaaaagtaattgca

SEQ ID NO: 17878 - RNA, 20 nt, synthetic construct
  source 1..20: mol_type = other RNA
gcctttaaaaaagtaattgc

SEQ ID NO: 17879 - RNA, 20 nt, synthetic construct
  source 1..20: mol_type = other RNA
ttaaaggcacttttactctt

SEQ ID NO: 17880 - RNA, 20 nt, synthetic construct
  source 1..20: mol_type = other RNA
gctagtaaatattagcaaaa

SEQ ID NO: 17881 - RNA, 20 nt, synthetic construct
  source 1..20: mol_type = other RNA
tagctttataaattacagta

SEQ ID NO: 17882 - RNA, 20 nt, synthetic construct
  source 1..20: mol_type = other RNA
aagtacatatattttgcaca

SEQ ID NO: 17883 - RNA, 20 nt, synthetic construct
  source 1..20: mol_type = other RNA
gttttatactgctaagtgct

SEQ ID NO: 17884 - RNA, 20 nt, synthetic construct
  source 1..20: mol_type = other RNA
tatactgctaagtgcttggt

SEQ ID NO: 17885 - RNA, 20 nt, synthetic construct
  source 1..20: mol_type = other RNA
atactgctaagtgcttggtt

SEQ ID NO: 17886 - RNA, 20 nt, synthetic construct
  source 1..20: mol_type = other RNA
tactgctaagtgcttggttg

SEQ ID NO: 17887 - RNA, 20 nt, synthetic construct
  source 1..20: mol_type = other RNA
tgctaagtgcttggttgggg

SEQ ID NO: 17888 - RNA, 20 nt, synthetic construct
  source 1..20: mol_type = other RNA
ggtgagatgatgattagatc

SEQ ID NO: 17889 - RNA, 20 nt, synthetic construct
  source 1..20: mol_type = other RNA
gtgagatgatgattagatca

SEQ ID NO: 17890 - RNA, 20 nt, synthetic construct
  source 1..20: mol_type = other RNA
tgagatgatgattagatcag

SEQ ID NO: 17891 - RNA, 20 nt, synthetic construct
  source 1..20: mol_type = other RNA
tgatgattagatcaggggtg

SEQ ID NO: 17892 - RNA, 20 nt, synthetic construct
  source 1..20: mol_type = other RNA
ggggtgaggctgagagactc

SEQ ID NO: 17893 - RNA, 20 nt, synthetic construct
  source 1..20: mol_type = other RNA
gggtgaggctgagagactct

SEQ ID NO: 17894 - RNA, 20 nt, synthetic construct
  source 1..20: mol_type = other RNA
ggctgagagactctgggttt

SEQ ID NO: 17895 - RNA, 20 nt, synthetic construct
  source 1..20: mol_type = other RNA
gctgagagactctgggttta

SEQ ID NO: 17896 - RNA, 20 nt, synthetic construct
  source 1..20: mol_type = other RNA
agccctgcctccatctccct

SEQ ID NO: 17897 - RNA, 20 nt, synthetic construct
  source 1..20: mol_type = other RNA
gccctgcctccatctccctt

SEQ ID NO: 17898 - RNA, 20 nt, synthetic construct
  source 1..20: mol_type = other RNA
acccaagggagatggaggca

SEQ ID NO: 17899 - RNA, 20 nt, synthetic construct
  source 1..20: mol_type = other RNA
tacccaagggagatggaggc

SEQ ID NO: 17900 - RNA, 20 nt, synthetic construct
  source 1..20: mol_type = other RNA
atctcccttgggtaaaatga

SEQ ID NO: 17901 - RNA, 20 nt, synthetic construct
  source 1..20: mol_type = other RNA
tctcccttgggtaaaatgaa

SEQ ID NO: 17902 - RNA, 20 nt, synthetic construct
  source 1..20: mol_type = other RNA
ttcattttacccaagggaga

SEQ ID NO: 17903 - RNA, 20 nt, synthetic construct
  source 1..20: mol_type = other RNA
cttgggtaaaatgaagggtg

SEQ ID NO: 17904 - RNA, 20 nt, synthetic construct
  source 1..20: mol_type = other RNA
ttgggtaaaatgaagggtgt

SEQ ID NO: 17905 - RNA, 20 nt, synthetic construct
  source 1..20: mol_type = other RNA
tgggtaaaatgaagggtgtg

SEQ ID NO: 17906 - RNA, 20 nt, synthetic construct
  source 1..20: mol_type = other RNA
acacccttcattttacccaa

SEQ ID NO: 17907 - RNA, 20 nt, synthetic construct
  source 1..20: mol_type = other RNA
cacacccttcattttaccca

SEQ ID NO: 17908 - RNA, 20 nt, synthetic construct
  source 1..20: mol_type = other RNA
tgtggggtaaaagatgcata

SEQ ID NO: 17909 - RNA, 20 nt, synthetic construct
  source 1..20: mol_type = other RNA
taggctgtcagagctagaaa

SEQ ID NO: 17910 - RNA, 20 nt, synthetic construct
  source 1..20: mol_type = other RNA
tacagggtgattggacttct

SEQ ID NO: 17911 - RNA, 20 nt, synthetic construct
  source 1..20: mol_type = other RNA
catatttattacagggtgat

SEQ ID NO: 17912 - RNA, 20 nt, synthetic construct
  source 1..20: mol_type = other RNA
ttcaacacatatttattaca

SEQ ID NO: 17913 - RNA, 20 nt, synthetic construct
  source 1..20: mol_type = other RNA
attcaacacatatttattac

SEQ ID NO: 17914 - RNA, 20 nt, synthetic construct
  source 1..20: mol_type = other RNA
atatgtgttgaatgaagaaa

SEQ ID NO: 17915 - RNA, 20 nt, synthetic construct
  source 1..20: mol_type = other RNA
tatgtgttgaatgaagaaat

SEQ ID NO: 17916 - RNA, 20 nt, synthetic construct
  source 1..20: mol_type = other RNA
attttaaaaaattgactacc

SEQ ID NO: 17917 - RNA, 20 nt, synthetic construct
  source 1..20: mol_type = other RNA
ttaaaaaattgactacctgg

SEQ ID NO: 17918 - RNA, 20 nt, synthetic construct
  source 1..20: mol_type = other RNA
gactacctggaggaatgatt

SEQ ID NO: 17919 - RNA, 20 nt, synthetic construct
  source 1..20: mol_type = other RNA
agattcctaatcattcctcc

SEQ ID NO: 17920 - RNA, 20 nt, synthetic construct
  source 1..20: mol_type = other RNA
atctaaatgaagccagccct

SEQ ID NO: 17921 - RNA, 20 nt, synthetic construct
  source 1..20: mol_type = other RNA
agccagccctcggtatctgc

SEQ ID NO: 17922 - RNA, 20 nt, synthetic construct
  source 1..20: mol_type = other RNA
aacctgcagataccgagggc

SEQ ID NO: 17923 - RNA, 20 nt, synthetic construct
  source 1..20: mol_type = other RNA
gagaaacctgcagataccga

SEQ ID NO: 17924 - RNA, 20 nt, synthetic construct
  source 1..20: mol_type = other RNA
tgagaaacctgcagataccg

SEQ ID NO: 17925 - RNA, 20 nt, synthetic construct
  source 1..20: mol_type = other RNA
atctgcaggtttctcatcca

SEQ ID NO: 17926 - RNA, 20 nt, synthetic construct
  source 1..20: mol_type = other RNA
tggattcaaccaactgcaaa

SEQ ID NO: 17927 - RNA, 20 nt, synthetic construct
  source 1..20: mol_type = other RNA
tttgcagttggttgaatcca

SEQ ID NO: 17928 - RNA, 20 nt, synthetic construct
  source 1..20: mol_type = other RNA
tcgtattttccatttgcagt

SEQ ID NO: 17929 - RNA, 20 nt, synthetic construct
  source 1..20: mol_type = other RNA
atacgattttttttaaaaaa

SEQ ID NO: 17930 - RNA, 20 nt, synthetic construct
  source 1..20: mol_type = other RNA
gattttttttaaaaaaagga

SEQ ID NO: 17931 - RNA, 20 nt, synthetic construct
  source 1..20: mol_type = other RNA
aagtctgtacatgttcaata

SEQ ID NO: 17932 - RNA, 20 nt, synthetic construct
  source 1..20: mol_type = other RNA
atgtagcatttacatttatt

SEQ ID NO: 17933 - RNA, 20 nt, synthetic construct
  source 1..20: mol_type = other RNA
attatttaattaaaatatac

SEQ ID NO: 17934 - RNA, 20 nt, synthetic construct
  source 1..20: mol_type = other RNA
atttaattaaaatatacagg

SEQ ID NO: 17935 - RNA, 20 nt, synthetic construct
  source 1..20: mol_type = other RNA
attctgtaccattttgtatc

SEQ ID NO: 17936 - RNA, 20 nt, synthetic construct
  source 1..20: mol_type = other RNA
ttctgtaccattttgtatca

SEQ ID NO: 17937 - RNA, 20 nt, synthetic construct
  source 1..20: mol_type = other RNA
ctcaattccctgatacaaaa

SEQ ID NO: 17938 - RNA, 20 nt, synthetic construct
  source 1..20: mol_type = other RNA
aattgagcatcttcagatgt

SEQ ID NO: 17939 - RNA, 20 nt, synthetic construct
  source 1..20: mol_type = other RNA
cttcagatgttggtatctgc

SEQ ID NO: 17940 - RNA, 20 nt, synthetic construct
  source 1..20: mol_type = other RNA
ttcagatgttggtatctgca

SEQ ID NO: 17941 - RNA, 20 nt, synthetic construct
  source 1..20: mol_type = other RNA
gttggtatctgcagggatcc

SEQ ID NO: 17942 - RNA, 20 nt, synthetic construct
  source 1..20: mol_type = other RNA
atctgcaggggtttggttcc

SEQ ID NO: 17943 - RNA, 20 nt, synthetic construct
  source 1..20: mol_type = other RNA
ccaaacccctgcagatacta

SEQ ID NO: 17944 - RNA, 20 nt, synthetic construct
  source 1..20: mol_type = other RNA
caaacccctgcagatactaa

SEQ ID NO: 17945 - RNA, 20 nt, synthetic construct
  source 1..20: mol_type = other RNA
ccttagtatctgcaggggtt

SEQ ID NO: 17946 - RNA, 20 nt, synthetic construct
  source 1..20: mol_type = other RNA
tcagcccttagtatctgcag

SEQ ID NO: 17947 - RNA, 20 nt, synthetic construct
  source 1..20: mol_type = other RNA
gtcagcccttagtatctgca

SEQ ID NO: 17948 - RNA, 20 nt, synthetic construct
  source 1..20: mol_type = other RNA
cgtcagcccttagtatctgc

SEQ ID NO: 17949 - RNA, 20 nt, synthetic construct
  source 1..20: mol_type = other RNA
atactaagggctgacgatct

SEQ ID NO: 17950 - RNA, 20 nt, synthetic construct
  source 1..20: mol_type = other RNA
gctgacgatctaggtaagac

SEQ ID NO: 17951 - RNA, 20 nt, synthetic construct
  source 1..20: mol_type = other RNA
gtaagactggatttaacagt

SEQ ID NO: 17952 - RNA, 20 nt, synthetic construct
  source 1..20: mol_type = other RNA
gttggaaaaaaaaaaaaaaa

SEQ ID NO: 17953 - RNA, 20 nt, synthetic construct
  source 1..20: mol_type = other RNA
tgttttaatttctacaggaa

SEQ ID NO: 17954 - RNA, 20 nt, synthetic construct
  source 1..20: mol_type = other RNA
tattttgttttaatttctac

SEQ ID NO: 17955 - RNA, 20 nt, synthetic construct
  source 1..20: mol_type = other RNA
ttaaaacaaaatacaaattg

SEQ ID NO: 17956 - RNA, 20 nt, synthetic construct
  source 1..20: mol_type = other RNA
ttgaggaagctctgctaccc

SEQ ID NO: 17957 - RNA, 20 nt, synthetic construct
  source 1..20: mol_type = other RNA
ctctgctacccaggctgtca

SEQ ID NO: 17958 - RNA, 20 nt, synthetic construct
  source 1..20: mol_type = other RNA
gttctctaccatgacagcct

SEQ ID NO: 17959 - RNA, 20 nt, synthetic construct
  source 1..20: mol_type = other RNA
agttctctaccatgacagcc

SEQ ID NO: 17960 - RNA, 20 nt, synthetic construct
  source 1..20: mol_type = other RNA
gaacttgaagaagacctgtt

SEQ ID NO: 17961 - RNA, 20 nt, synthetic construct
  source 1..20: mol_type = other RNA
ttgaagaagacctgtttgga

SEQ ID NO: 17962 - RNA, 20 nt, synthetic construct
  source 1..20: mol_type = other RNA
gacctgtttggatggacacc

SEQ ID NO: 17963 - RNA, 20 nt, synthetic construct
  source 1..20: mol_type = other RNA
aaccaggtgtccatccaaac

SEQ ID NO: 17964 - RNA, 20 nt, synthetic construct
  source 1..20: mol_type = other RNA
gacacctggtttcaaaagtc

SEQ ID NO: 17965 - RNA, 20 nt, synthetic construct
  source 1..20: mol_type = other RNA
ctggtttcaaaagtcaggtg

SEQ ID NO: 17966 - RNA, 20 nt, synthetic construct
  source 1..20: mol_type = other RNA
cacacctgacttttgaaacc

SEQ ID NO: 17967 - RNA, 20 nt, synthetic construct
  source 1..20: mol_type = other RNA
caggtgtggagactgttaaa

SEQ ID NO: 17968 - RNA, 20 nt, synthetic construct
  source 1..20: mol_type = other RNA
aggtgtggagactgttaaat

SEQ ID NO: 17969 - RNA, 20 nt, synthetic construct
  source 1..20: mol_type = other RNA
tgtggagactgttaaatggg

SEQ ID NO: 17970 - RNA, 20 nt, synthetic construct
  source 1..20: mol_type = other RNA
gtggagactgttaaatggga

SEQ ID NO: 17971 - RNA, 20 nt, synthetic construct
  source 1..20: mol_type = other RNA
cctcatccataaatgatttc

SEQ ID NO: 17972 - RNA, 20 nt, synthetic construct
  source 1..20: mol_type = other RNA
ccagaaatcatttatggatg

SEQ ID NO: 17973 - RNA, 20 nt, synthetic construct
  source 1..20: mol_type = other RNA
acgttgccagaaatcattta

SEQ ID NO: 17974 - RNA, 20 nt, synthetic construct
  source 1..20: mol_type = other RNA
tttctggcaacgtcttcttc

SEQ ID NO: 17975 - RNA, 20 nt, synthetic construct
  source 1..20: mol_type = other RNA
ctggcaacgtcttcttcagg

SEQ ID NO: 17976 - RNA, 20 nt, synthetic construct
  source 1..20: mol_type = other RNA
gacgtctttttaatgttact

SEQ ID NO: 17977 - RNA, 20 nt, synthetic construct
  source 1..20: mol_type = other RNA
acgtctttttaatgttactt

SEQ ID NO: 17978 - RNA, 20 nt, synthetic construct
  source 1..20: mol_type = other RNA
cgtctttttaatgttacttg

SEQ ID NO: 17979 - RNA, 20 nt, synthetic construct
  source 1..20: mol_type = other RNA
ctttttaatgttacttgggg

SEQ ID NO: 17980 - RNA, 20 nt, synthetic construct
  source 1..20: mol_type = other RNA
tttttaatgttacttgggga

SEQ ID NO: 17981 - RNA, 20 nt, synthetic construct
  source 1..20: mol_type = other RNA
tggggagggagtgctcatta

SEQ ID NO: 17982 - RNA, 20 nt, synthetic construct
  source 1..20: mol_type = other RNA
ggggagggagtgctcattaa

SEQ ID NO: 17983 - RNA, 20 nt, synthetic construct
  source 1..20: mol_type = other RNA
agtgctcattaagggatgcc

SEQ ID NO: 17984 - RNA, 20 nt, synthetic construct
  source 1..20: mol_type = other RNA
gtgctcattaagggatgcca

SEQ ID NO: 17985 - RNA, 20 nt, synthetic construct
  source 1..20: mol_type = other RNA
agggatgccagggccagctc

SEQ ID NO: 17986 - RNA, 20 nt, synthetic construct
  source 1..20: mol_type = other RNA
gatgccagggccagctctgg

SEQ ID NO: 17987 - RNA, 20 nt, synthetic construct
  source 1..20: mol_type = other RNA
gggccagctctggtggttcc

SEQ ID NO: 17988 - RNA, 20 nt, synthetic construct
  source 1..20: mol_type = other RNA
ggccagctctggtggttcct

SEQ ID NO: 17989 - RNA, 20 nt, synthetic construct
  source 1..20: mol_type = other RNA
gccagctctggtggttcctg

SEQ ID NO: 17990 - RNA, 20 nt, synthetic construct
  source 1..20: mol_type = other RNA
agctctggtggttcctgggg

SEQ ID NO: 17991 - RNA, 20 nt, synthetic construct
  source 1..20: mol_type = other RNA
tccccaggaaccaccagagc

SEQ ID NO: 17992 - RNA, 20 nt, synthetic construct
  source 1..20: mol_type = other RNA
gggaaggacgcagcctcccc

SEQ ID NO: 17993 - RNA, 20 nt, synthetic construct
  source 1..20: mol_type = other RNA
ccctgcttctgcatgtcatg

SEQ ID NO: 17994 - RNA, 20 nt, synthetic construct
  source 1..20: mol_type = other RNA
atgacatgcagaagcaggga

SEQ ID NO: 17995 - RNA, 20 nt, synthetic construct
  source 1..20: mol_type = other RNA
cctcatgacatgcagaagca

SEQ ID NO: 17996 - RNA, 20 nt, synthetic construct
  source 1..20: mol_type = other RNA
gcctcatgacatgcagaagc

SEQ ID NO: 17997 - RNA, 20 nt, synthetic construct
  source 1..20: mol_type = other RNA
tctgcatgtcatgaggcagc

SEQ ID NO: 17998 - RNA, 20 nt, synthetic construct
  source 1..20: mol_type = other RNA
catgtcatgaggcagcagga

SEQ ID NO: 17999 - RNA, 20 nt, synthetic construct
  source 1..20: mol_type = other RNA
tcccctgcacctgtctgtcc

SEQ ID NO: 18000 - RNA, 20 nt, synthetic construct
  source 1..20: mol_type = other RNA
gccaggacagacaggtgcag

SEQ ID NO: 18001 - RNA, 20 nt, synthetic construct
  source 1..20: mol_type = other RNA
agccaggacagacaggtgca

SEQ ID NO: 18002 - RNA, 20 nt, synthetic construct
  source 1..20: mol_type = other RNA
gagccaggacagacaggtgc

SEQ ID NO: 18003 - RNA, 20 nt, synthetic construct
  source 1..20: mol_type = other RNA
ctgtctgtcctggctccctc

SEQ ID NO: 18004 - RNA, 20 nt, synthetic construct
  source 1..20: mol_type = other RNA
tgtctgtcctggctccctct

SEQ ID NO: 18005 - RNA, 20 nt, synthetic construct
  source 1..20: mol_type = other RNA
cagagggagccaggacagac

SEQ ID NO: 18006 - RNA, 20 nt, synthetic construct
  source 1..20: mol_type = other RNA
ggggctacccagagggagcc

SEQ ID NO: 18007 - RNA, 20 nt, synthetic construct
  source 1..20: mol_type = other RNA
acagtagggggctacccaga

SEQ ID NO: 18008 - RNA, 20 nt, synthetic construct
  source 1..20: mol_type = other RNA
aacagtagggggctacccag

SEQ ID NO: 18009 - RNA, 20 nt, synthetic construct
  source 1..20: mol_type = other RNA
ctgaagcacagaacagtagg

SEQ ID NO: 18010 - RNA, 20 nt, synthetic construct
  source 1..20: mol_type = other RNA
gctgaagcacagaacagtag

SEQ ID NO: 18011 - RNA, 20 nt, synthetic construct
  source 1..20: mol_type = other RNA
tgctgaagcacagaacagta

SEQ ID NO: 18012 - RNA, 20 nt, synthetic construct
  source 1..20: mol_type = other RNA
gtgctgaagcacagaacagt

SEQ ID NO: 18013 - RNA, 20 nt, synthetic construct
  source 1..20: mol_type = other RNA
ttctgtgcttcagcacagcc

SEQ ID NO: 18014 - RNA, 20 nt, synthetic construct
  source 1..20: mol_type = other RNA
gcacagcctggtttgtcaag

SEQ ID NO: 18015 - RNA, 20 nt, synthetic construct
  source 1..20: mol_type = other RNA
tttgtcaagaggcacatagt

SEQ ID NO: 18016 - RNA, 20 nt, synthetic construct
  source 1..20: mol_type = other RNA
ttgtcaagaggcacatagtt

SEQ ID NO: 18017 - RNA, 20 nt, synthetic construct
  source 1..20: mol_type = other RNA
tgtcaagaggcacatagttg

SEQ ID NO: 18018 - RNA, 20 nt, synthetic construct
  source 1..20: mol_type = other RNA
aagaggcacatagttggggc

SEQ ID NO: 18019 - RNA, 20 nt, synthetic construct
  source 1..20: mol_type = other RNA
agaggcacatagttggggct

SEQ ID NO: 18020 - RNA, 20 nt, synthetic construct
  source 1..20: mol_type = other RNA
atagttggggctgggctgca

SEQ ID NO: 18021 - RNA, 20 nt, synthetic construct
  source 1..20: mol_type = other RNA
ggggctgggctgcatggcac

SEQ ID NO: 18022 - RNA, 20 nt, synthetic construct
  source 1..20: mol_type = other RNA
gggctgggctgcatggcaca

SEQ ID NO: 18023 - RNA, 20 nt, synthetic construct
  source 1..20: mol_type = other RNA
ggctgggctgcatggcacag

SEQ ID NO: 18024 - RNA, 20 nt, synthetic construct
  source 1..20: mol_type = other RNA
acaggggcttatgtgcctgc

SEQ ID NO: 18025 - RNA, 20 nt, synthetic construct
  source 1..20: mol_type = other RNA
ctgaaaattaaataaccagc

SEQ ID NO: 18026 - RNA, 20 nt, synthetic construct
  source 1..20: mol_type = other RNA
aaaatattaaagaaaactta

SEQ ID NO: 18027 - RNA, 20 nt, synthetic construct
  source 1..20: mol_type = other RNA
tttctttaatattttcctgt

SEQ ID NO: 18028 - RNA, 20 nt, synthetic construct
  source 1..20: mol_type = other RNA
ttttcctgttggctatttaa

SEQ ID NO: 18029 - RNA, 20 nt, synthetic construct
  source 1..20: mol_type = other RNA
tgttggctatttaaaggttt

SEQ ID NO: 18030 - RNA, 20 nt, synthetic construct
  source 1..20: mol_type = other RNA
aaaacctttaaatagccaac

SEQ ID NO: 18031 - RNA, 20 nt, synthetic construct
  source 1..20: mol_type = other RNA
tgtcatcttgattgtagata

SEQ ID NO: 18032 - RNA, 20 nt, synthetic construct
  source 1..20: mol_type = other RNA
gaattatcttatttataaca

SEQ ID NO: 18033 - RNA, 20 nt, synthetic construct
  source 1..20: mol_type = other RNA
cacatatttatttggaggtg

SEQ ID NO: 18034 - RNA, 20 nt, synthetic construct
  source 1..20: mol_type = other RNA
acacacacatatttatttgg

SEQ ID NO: 18035 - RNA, 20 nt, synthetic construct
  source 1..20: mol_type = other RNA
cagacacacacatatttatt

SEQ ID NO: 18036 - RNA, 20 nt, synthetic construct
  source 1..20: mol_type = other RNA
tgtgtgtgtatatatgtatg

SEQ ID NO: 18037 - RNA, 20 nt, synthetic construct
  source 1..20: mol_type = other RNA
gtgtgtatatatgtatgtgg

SEQ ID NO: 18038 - RNA, 20 nt, synthetic construct
  source 1..20: mol_type = other RNA
tatatatgtatgtggcggag

SEQ ID NO: 18039 - RNA, 20 nt, synthetic construct
  source 1..20: mol_type = other RNA
atatatgtatgtggcggaga

SEQ ID NO: 18040 - RNA, 20 nt, synthetic construct
  source 1..20: mol_type = other RNA
tgtggcggagagggagagag

SEQ ID NO: 18041 - RNA, 20 nt, synthetic construct
  source 1..20: mol_type = other RNA
gtggcggagagggagagagt

SEQ ID NO: 18042 - RNA, 20 nt, synthetic construct
  source 1..20: mol_type = other RNA
tggcggagagggagagagtg

SEQ ID NO: 18043 - RNA, 20 nt, synthetic construct
  source 1..20: mol_type = other RNA
ggagagggagagagtgggga

SEQ ID NO: 18044 - RNA, 20 nt, synthetic construct
  source 1..20: mol_type = other RNA
cagtgttatcatacatagag

SEQ ID NO: 18045 - RNA, 20 nt, synthetic construct
  source 1..20: mol_type = other RNA
taaagctgacagtgagggat

SEQ ID NO: 18046 - RNA, 20 nt, synthetic construct
  source 1..20: mol_type = other RNA
cctcactgtcagctttataa

SEQ ID NO: 18047 - RNA, 20 nt, synthetic construct
  source 1..20: mol_type = other RNA
ctttataaagctgacagtga

SEQ ID NO: 18048 - RNA, 20 nt, synthetic construct
  source 1..20: mol_type = other RNA
cctttataaagctgacagtg

SEQ ID NO: 18049 - RNA, 20 nt, synthetic construct
  source 1..20: mol_type = other RNA
ataaaacattcttctgtgga

SEQ ID NO: 18050 - RNA, 20 nt, synthetic construct
  source 1..20: mol_type = other RNA
gaagaatgttttataagact

SEQ ID NO: 18051 - RNA, 20 nt, synthetic construct
  source 1..20: mol_type = other RNA
aggaaaacacgttgaaaact

SEQ ID NO: 18052 - RNA, 20 nt, synthetic construct
  source 1..20: mol_type = other RNA
atatgttgttactgttgcta

SEQ ID NO: 18053 - RNA, 20 nt, synthetic construct
  source 1..20: mol_type = other RNA
ttttctccttagaataattt

SEQ ID NO: 18054 - RNA, 20 nt, synthetic construct
  source 1..20: mol_type = other RNA
aaaaatcctaaattattcta

SEQ ID NO: 18055 - RNA, 20 nt, synthetic construct
  source 1..20: mol_type = other RNA
tgccaaatgctgtagataaa

SEQ ID NO: 18056 - RNA, 20 nt, synthetic construct
  source 1..20: mol_type = other RNA
ggccatttatctacagcatt

SEQ ID NO: 18057 - RNA, 20 nt, synthetic construct
  source 1..20: mol_type = other RNA
gccagattcttcctatccct

SEQ ID NO: 18058 - RNA, 20 nt, synthetic construct
  source 1..20: mol_type = other RNA
tcctagggataggaagaatc

SEQ ID NO: 18059 - RNA, 20 nt, synthetic construct
  source 1..20: mol_type = other RNA
aataaaggaatcctagggat

SEQ ID NO: 18060 - RNA, 20 nt, synthetic construct
  source 1..20: mol_type = other RNA
aaaataataaaggaatccta

SEQ ID NO: 18061 - RNA, 20 nt, synthetic construct
  source 1..20: mol_type = other RNA
aaaaataataaaggaatcct

SEQ ID NO: 18062 - RNA, 20 nt, synthetic construct
  source 1..20: mol_type = other RNA
tctgtgaaaaaaaataataa

SEQ ID NO: 18063 - RNA, 20 nt, synthetic construct
  source 1..20: mol_type = other RNA
tttcacagattttgagaaca

SEQ ID NO: 18064 - RNA, 20 nt, synthetic construct
  source 1..20: mol_type = other RNA
ttcacagattttgagaacaa

SEQ ID NO: 18065 - RNA, 20 nt, synthetic construct
  source 1..20: mol_type = other RNA
tcacagattttgagaacaag

SEQ ID NO: 18066 - RNA, 20 nt, synthetic construct
  source 1..20: mol_type = other RNA
cacagattttgagaacaagg

SEQ ID NO: 18067 - RNA, 20 nt, synthetic construct
  source 1..20: mol_type = other RNA
aacaagggggagagatagta

SEQ ID NO: 18068 - RNA, 20 nt, synthetic construct
  source 1..20: mol_type = other RNA
acacagttctataagattaa

SEQ ID NO: 18069 - RNA, 20 nt, synthetic construct
  source 1..20: mol_type = other RNA
aattcctgcttgtttgaaca

SEQ ID NO: 18070 - RNA, 20 nt, synthetic construct
  source 1..20: mol_type = other RNA
gttcaaacaagcaggaattt

SEQ ID NO: 18071 - RNA, 20 nt, synthetic construct
  source 1..20: mol_type = other RNA
tgttcaaacaagcaggaatt

SEQ ID NO: 18072 - RNA, 20 nt, synthetic construct
  source 1..20: mol_type = other RNA
gatgccatgttcaaacaagc

SEQ ID NO: 18073 - RNA, 20 nt, synthetic construct
  source 1..20: mol_type = other RNA
catggcatcttcatagattc

SEQ ID NO: 18074 - RNA, 20 nt, synthetic construct
  source 1..20: mol_type = other RNA
gattcactaccctctatagc

SEQ ID NO: 18075 - RNA, 20 nt, synthetic construct
  source 1..20: mol_type = other RNA
tttcaagatccagctataga

SEQ ID NO: 18076 - RNA, 20 nt, synthetic construct
  source 1..20: mol_type = other RNA
ttttcaagatccagctatag

SEQ ID NO: 18077 - RNA, 20 nt, synthetic construct
  source 1..20: mol_type = other RNA
gctggatcttgaaaattatc

SEQ ID NO: 18078 - RNA, 20 nt, synthetic construct
  source 1..20: mol_type = other RNA
cagataattttgcatctgct

SEQ ID NO: 18079 - RNA, 20 nt, synthetic construct
  source 1..20: mol_type = other RNA
caagcagatgcaaaattatc

SEQ ID NO: 18080 - RNA, 20 nt, synthetic construct
  source 1..20: mol_type = other RNA
attgtagactgagatgtgag

SEQ ID NO: 18081 - RNA, 20 nt, synthetic construct
  source 1..20: mol_type = other RNA
gtagactgagatgtgagtgg

SEQ ID NO: 18082 - RNA, 20 nt, synthetic construct
  source 1..20: mol_type = other RNA
gccaaccaagaagtatttat

SEQ ID NO: 18083 - RNA, 20 nt, synthetic construct
  source 1..20: mol_type = other RNA
tccgataaatacttcttggt

SEQ ID NO: 18084 - RNA, 20 nt, synthetic construct
  source 1..20: mol_type = other RNA
agtgtccgataaatacttct

SEQ ID NO: 18085 - RNA, 20 nt, synthetic construct
  source 1..20: mol_type = other RNA
gtatttatcggacacttact

SEQ ID NO: 18086 - RNA, 20 nt, synthetic construct
  source 1..20: mol_type = other RNA
cggacacttactaggtgcct

SEQ ID NO: 18087 - RNA, 20 nt, synthetic construct
  source 1..20: mol_type = other RNA
ggtgcctaggattgtatcag

SEQ ID NO: 18088 - RNA, 20 nt, synthetic construct
  source 1..20: mol_type = other RNA
gtgcctaggattgtatcaga

SEQ ID NO: 18089 - RNA, 20 nt, synthetic construct
  source 1..20: mol_type = other RNA
attccctctgatacaatcct

SEQ ID NO: 18090 - RNA, 20 nt, synthetic construct
  source 1..20: mol_type = other RNA
cgttaaaactaggtagggca

SEQ ID NO: 18091 - RNA, 20 nt, synthetic construct
  source 1..20: mol_type = other RNA
tcgttaaaactaggtagggc

SEQ ID NO: 18092 - RNA, 20 nt, synthetic construct
  source 1..20: mol_type = other RNA
tctgtcgttaaaactaggta

SEQ ID NO: 18093 - RNA, 20 nt, synthetic construct
  source 1..20: mol_type = other RNA
ttctgtcgttaaaactaggt

SEQ ID NO: 18094 - RNA, 20 nt, synthetic construct
  source 1..20: mol_type = other RNA
gatattctgtcgttaaaact

SEQ ID NO: 18095 - RNA, 20 nt, synthetic construct
  source 1..20: mol_type = other RNA
aacgacagaatatctattaa

SEQ ID NO: 18096 - RNA, 20 nt, synthetic construct
  source 1..20: mol_type = other RNA
attaaaggctacttagctga

SEQ ID NO: 18097 - RNA, 20 nt, synthetic construct
  source 1..20: mol_type = other RNA
ttaaaggctacttagctgaa

SEQ ID NO: 18098 - RNA, 20 nt, synthetic construct
  source 1..20: mol_type = other RNA
ggctacttagctgaagggta

SEQ ID NO: 18099 - RNA, 20 nt, synthetic construct
  source 1..20: mol_type = other RNA
gctacttagctgaagggtaa

SEQ ID NO: 18100 - RNA, 20 nt, synthetic construct
  source 1..20: mol_type = other RNA
agctgaagggtaagggtgac

SEQ ID NO: 18101 - RNA, 20 nt, synthetic construct
  source 1..20: mol_type = other RNA
agggtaagggtgacaggtct

SEQ ID NO: 18102 - RNA, 20 nt, synthetic construct
  source 1..20: mol_type = other RNA
gggtaagggtgacaggtcta

SEQ ID NO: 18103 - RNA, 20 nt, synthetic construct
  source 1..20: mol_type = other RNA
ggtaagggtgacaggtctag

SEQ ID NO: 18104 - RNA, 20 nt, synthetic construct
  source 1..20: mol_type = other RNA
gacaggtctaggggaagctt

SEQ ID NO: 18105 - RNA, 20 nt, synthetic construct
  source 1..20: mol_type = other RNA
acaggtctaggggaagcttt

SEQ ID NO: 18106 - RNA, 20 nt, synthetic construct
  source 1..20: mol_type = other RNA
ggtctaggggaagctttggg

SEQ ID NO: 18107 - RNA, 20 nt, synthetic construct
  source 1..20: mol_type = other RNA
ctaggggaagctttgggagg

SEQ ID NO: 18108 - RNA, 20 nt, synthetic construct
  source 1..20: mol_type = other RNA
gtgtgctgtgacagaaaaag

SEQ ID NO: 18109 - RNA, 20 nt, synthetic construct
  source 1..20: mol_type = other RNA
gacagaaaaagtggcagagt

SEQ ID NO: 18110 - RNA, 20 nt, synthetic construct
  source 1..20: mol_type = other RNA
acagaaaaagtggcagagta

SEQ ID NO: 18111 - RNA, 20 nt, synthetic construct
  source 1..20: mol_type = other RNA
cagaaacagggctagaatgc

SEQ ID NO: 18112 - RNA, 20 nt, synthetic construct
  source 1..20: mol_type = other RNA
cagagcaagtgacagaaaca

SEQ ID NO: 18113 - RNA, 20 nt, synthetic construct
  source 1..20: mol_type = other RNA
acagagcaagtgacagaaac

SEQ ID NO: 18114 - RNA, 20 nt, synthetic construct
  source 1..20: mol_type = other RNA
ggaggaaactaaagctcaag

SEQ ID NO: 18115 - RNA, 20 nt, synthetic construct
  source 1..20: mol_type = other RNA
ttcctcctctgcataatgag

SEQ ID NO: 18116 - RNA, 20 nt, synthetic construct
  source 1..20: mol_type = other RNA
tcctcctctgcataatgaga

SEQ ID NO: 18117 - RNA, 20 nt, synthetic construct
  source 1..20: mol_type = other RNA
accctctcattatgcagagg

SEQ ID NO: 18118 - RNA, 20 nt, synthetic construct
  source 1..20: mol_type = other RNA
ctaaccctctcattatgcag

SEQ ID NO: 18119 - RNA, 20 nt, synthetic construct
  source 1..20: mol_type = other RNA
ggttagactactgaattgta

SEQ ID NO: 18120 - RNA, 20 nt, synthetic construct
  source 1..20: mol_type = other RNA
gttagactactgaattgtat

SEQ ID NO: 18121 - RNA, 20 nt, synthetic construct
  source 1..20: mol_type = other RNA
gggaaaaaaatacaaattcc

SEQ ID NO: 18122 - RNA, 20 nt, synthetic construct
  source 1..20: mol_type = other RNA
ggaaaaaaatacaaattcct

SEQ ID NO: 18123 - RNA, 20 nt, synthetic construct
  source 1..20: mol_type = other RNA
aatacaaattcctgggtcct

SEQ ID NO: 18124 - RNA, 20 nt, synthetic construct
  source 1..20: mol_type = other RNA
gcaggcatggcctaggaccc

SEQ ID NO: 18125 - RNA, 20 nt, synthetic construct
  source 1..20: mol_type = other RNA
ggattcagcaggcatggcct

SEQ ID NO: 18126 - RNA, 20 nt, synthetic construct
  source 1..20: mol_type = other RNA
cctgctgaatccgactgttc

SEQ ID NO: 18127 - RNA, 20 nt, synthetic construct
  source 1..20: mol_type = other RNA
cctgaacagtcggattcagc

SEQ ID NO: 18128 - RNA, 20 nt, synthetic construct
  source 1..20: mol_type = other RNA
gaatccgactgttcaggaag

SEQ ID NO: 18129 - RNA, 20 nt, synthetic construct
  source 1..20: mol_type = other RNA
gactgttcaggaagaggcct

SEQ ID NO: 18130 - RNA, 20 nt, synthetic construct
  source 1..20: mol_type = other RNA
taggcctcttcctgaacagt

SEQ ID NO: 18131 - RNA, 20 nt, synthetic construct
  source 1..20: mol_type = other RNA
agaggcctaggaaatctgtg

SEQ ID NO: 18132 - RNA, 20 nt, synthetic construct
  source 1..20: mol_type = other RNA
gaggcctaggaaatctgtga

SEQ ID NO: 18133 - RNA, 20 nt, synthetic construct
  source 1..20: mol_type = other RNA
gattccctcacagatttcct

SEQ ID NO: 18134 - RNA, 20 nt, synthetic construct
  source 1..20: mol_type = other RNA
aaatctgtgagggaatcccc

SEQ ID NO: 18135 - RNA, 20 nt, synthetic construct
  source 1..20: mol_type = other RNA
aatctgtgagggaatcccca

SEQ ID NO: 18136 - RNA, 20 nt, synthetic construct
  source 1..20: mol_type = other RNA
atctgtgagggaatccccag

SEQ ID NO: 18137 - RNA, 20 nt, synthetic construct
  source 1..20: mol_type = other RNA
ctggtcacgagattcccctg

SEQ ID NO: 18138 - RNA, 20 nt, synthetic construct
  source 1..20: mol_type = other RNA
gctggtcacgagattcccct

SEQ ID NO: 18139 - RNA, 20 nt, synthetic construct
  source 1..20: mol_type = other RNA
ggctggtcacgagattcccc

SEQ ID NO: 18140 - RNA, 20 nt, synthetic construct
  source 1..20: mol_type = other RNA
caggtgtgaaatctgctaac

SEQ ID NO: 18141 - RNA, 20 nt, synthetic construct
  source 1..20: mol_type = other RNA
cagttagcagatttcacacc

SEQ ID NO: 18142 - RNA, 20 nt, synthetic construct
  source 1..20: mol_type = other RNA
cttcactttttgtgattttg

SEQ ID NO: 18143 - RNA, 20 nt, synthetic construct
  source 1..20: mol_type = other RNA
cacaaaatcacaaaaagtga

SEQ ID NO: 18144 - RNA, 20 nt, synthetic construct
  source 1..20: mol_type = other RNA
tgtattattctacgtaaatg

SEQ ID NO: 18145 - RNA, 20 nt, synthetic construct
  source 1..20: mol_type = other RNA
gtattattctacgtaaatgt

SEQ ID NO: 18146 - RNA, 20 nt, synthetic construct
  source 1..20: mol_type = other RNA
tctacgtaaatgtgggtact

SEQ ID NO: 18147 - RNA, 20 nt, synthetic construct
  source 1..20: mol_type = other RNA
acctgctgtttgtttcctag

SEQ ID NO: 18148 - RNA, 20 nt, synthetic construct
  source 1..20: mol_type = other RNA
acctctaggaaacaaacagc

SEQ ID NO: 18149 - RNA, 20 nt, synthetic construct
  source 1..20: mol_type = other RNA
taaagactactaacacctct

SEQ ID NO: 18150 - RNA, 20 nt, synthetic construct
  source 1..20: mol_type = other RNA
aaatacaagtaagacttaag

SEQ ID NO: 18151 - RNA, 20 nt, synthetic construct
  source 1..20: mol_type = other RNA
gatatttgatgttatttacc

SEQ ID NO: 18152 - RNA, 20 nt, synthetic construct
  source 1..20: mol_type = other RNA
aaaaggggaagaaaatatcc

SEQ ID NO: 18153 - RNA, 20 nt, synthetic construct
  source 1..20: mol_type = other RNA
ttccccttttatttatttag

SEQ ID NO: 18154 - RNA, 20 nt, synthetic construct
  source 1..20: mol_type = other RNA
ttcctctaaataaataaaag

SEQ ID NO: 18155 - RNA, 20 nt, synthetic construct
  source 1..20: mol_type = other RNA
tttcctctaaataaataaaa

SEQ ID NO: 18156 - RNA, 20 nt, synthetic construct
  source 1..20: mol_type = other RNA
atttcctctaaataaataaa

SEQ ID NO: 18157 - RNA, 20 nt, synthetic construct
  source 1..20: mol_type = other RNA
ttagaggaaattgagattct

SEQ ID NO: 18158 - RNA, 20 nt, synthetic construct
  source 1..20: mol_type = other RNA
aaaatgaaaacaaaattcta

SEQ ID NO: 18159 - RNA, 20 nt, synthetic construct
  source 1..20: mol_type = other RNA
tttcattataaagtagcaaa

SEQ ID NO: 18160 - RNA, 20 nt, synthetic construct
  source 1..20: mol_type = other RNA
atgaaaatttaaaaattata

SEQ ID NO: 18161 - RNA, 20 nt, synthetic construct
  source 1..20: mol_type = other RNA
tgaaaatttaaaaattatat

SEQ ID NO: 18162 - RNA, 20 nt, synthetic construct
  source 1..20: mol_type = other RNA
tatatgggaagatttttctc

SEQ ID NO: 18163 - RNA, 20 nt, synthetic construct
  source 1..20: mol_type = other RNA
atatgggaagatttttctct

SEQ ID NO: 18164 - RNA, 20 nt, synthetic construct
  source 1..20: mol_type = other RNA
aatccttgtcataaagtaag

SEQ ID NO: 18165 - RNA, 20 nt, synthetic construct
  source 1..20: mol_type = other RNA
agacctcttactttatgaca

SEQ ID NO: 18166 - RNA, 20 nt, synthetic construct
  source 1..20: mol_type = other RNA
gtaagaggtctttttaaagt

SEQ ID NO: 18167 - RNA, 20 nt, synthetic construct
  source 1..20: mol_type = other RNA
gaggtctttttaaagtaggt

SEQ ID NO: 18168 - RNA, 20 nt, synthetic construct
  source 1..20: mol_type = other RNA
tttaaagtaggtaggctata

SEQ ID NO: 18169 - RNA, 20 nt, synthetic construct
  source 1..20: mol_type = other RNA
ggagtattattttaaattac

SEQ ID NO: 18170 - RNA, 20 nt, synthetic construct
  source 1..20: mol_type = other RNA
aaaataatactcctttctct

SEQ ID NO: 18171 - RNA, 20 nt, synthetic construct
  source 1..20: mol_type = other RNA
aaataatactcctttctcta

SEQ ID NO: 18172 - RNA, 20 nt, synthetic construct
  source 1..20: mol_type = other RNA
atactcctttctctagggtt

SEQ ID NO: 18173 - RNA, 20 nt, synthetic construct
  source 1..20: mol_type = other RNA
ttgcaccaaaccctagagaa

SEQ ID NO: 18174 - RNA, 20 nt, synthetic construct
  source 1..20: mol_type = other RNA
tcaaatgttatcttcattaa

SEQ ID NO: 18175 - RNA, 20 nt, synthetic construct
  source 1..20: mol_type = other RNA
acatttgaattccccaaagc

SEQ ID NO: 18176 - RNA, 20 nt, synthetic construct
  source 1..20: mol_type = other RNA
tgaattccccaaagcaggtg

SEQ ID NO: 18177 - RNA, 20 nt, synthetic construct
  source 1..20: mol_type = other RNA
ccccaaagcaggtgaggagt

SEQ ID NO: 18178 - RNA, 20 nt, synthetic construct
  source 1..20: mol_type = other RNA
cccaaagcaggtgaggagtc

SEQ ID NO: 18179 - RNA, 20 nt, synthetic construct
  source 1..20: mol_type = other RNA
ccaaagcaggtgaggagtcg

SEQ ID NO: 18180 - RNA, 20 nt, synthetic construct
  source 1..20: mol_type = other RNA
ccgactcctcacctgctttg

SEQ ID NO: 18181 - RNA, 20 nt, synthetic construct
  source 1..20: mol_type = other RNA
cccgactcctcacctgcttt

SEQ ID NO: 18182 - RNA, 20 nt, synthetic construct
  source 1..20: mol_type = other RNA
ccccgactcctcacctgctt

SEQ ID NO: 18183 - RNA, 20 nt, synthetic construct
  source 1..20: mol_type = other RNA
atgaaaactcactgcaaaag

SEQ ID NO: 18184 - RNA, 20 nt, synthetic construct
  source 1..20: mol_type = other RNA
aaaactcactgcaaaagagg

SEQ ID NO: 18185 - RNA, 20 nt, synthetic construct
  source 1..20: mol_type = other RNA
cactgcaaaagaggaggcag

SEQ ID NO: 18186 - RNA, 20 nt, synthetic construct
  source 1..20: mol_type = other RNA
aaagaggaggcagaggaaga

SEQ ID NO: 18187 - RNA, 20 nt, synthetic construct
  source 1..20: mol_type = other RNA
ccccttaaagcagatgtgtg

SEQ ID NO: 18188 - RNA, 20 nt, synthetic construct
  source 1..20: mol_type = other RNA
cccttaaagcagatgtgtgt

SEQ ID NO: 18189 - RNA, 20 nt, synthetic construct
  source 1..20: mol_type = other RNA
ccttaaagcagatgtgtgtg

SEQ ID NO: 18190 - RNA, 20 nt, synthetic construct
  source 1..20: mol_type = other RNA
ccacacacatctgctttaag

SEQ ID NO: 18191 - RNA, 20 nt, synthetic construct
  source 1..20: mol_type = other RNA
cccacacacatctgctttaa

SEQ ID NO: 18192 - RNA, 20 nt, synthetic construct
  source 1..20: mol_type = other RNA
ccccacacacatctgcttta

SEQ ID NO: 18193 - RNA, 20 nt, synthetic construct
  source 1..20: mol_type = other RNA
tgtggggccttatgaagacc

SEQ ID NO: 18194 - RNA, 20 nt, synthetic construct
  source 1..20: mol_type = other RNA
ttatgaagaccaggattctg

SEQ ID NO: 18195 - RNA, 20 nt, synthetic construct
  source 1..20: mol_type = other RNA
tatgaagaccaggattctgc

SEQ ID NO: 18196 - RNA, 20 nt, synthetic construct
  source 1..20: mol_type = other RNA
gcagaatcctggtcttcata

SEQ ID NO: 18197 - RNA, 20 nt, synthetic construct
  source 1..20: mol_type = other RNA
accaggattctgcgggtgtc

SEQ ID NO: 18198 - RNA, 20 nt, synthetic construct
  source 1..20: mol_type = other RNA
ccaggattctgcgggtgtca

SEQ ID NO: 18199 - RNA, 20 nt, synthetic construct
  source 1..20: mol_type = other RNA
caggattctgcgggtgtcag

SEQ ID NO: 18200 - RNA, 20 nt, synthetic construct
  source 1..20: mol_type = other RNA
ccctgacacccgcagaatcc

SEQ ID NO: 18201 - RNA, 20 nt, synthetic construct
  source 1..20: mol_type = other RNA
tgcccctcttgacagagact

SEQ ID NO: 18202 - RNA, 20 nt, synthetic construct
  source 1..20: mol_type = other RNA
gcccctcttgacagagacta

SEQ ID NO: 18203 - RNA, 20 nt, synthetic construct
  source 1..20: mol_type = other RNA
accctagtctctgtcaagag

SEQ ID NO: 18204 - RNA, 20 nt, synthetic construct
  source 1..20: mol_type = other RNA
aaccctagtctctgtcaaga

SEQ ID NO: 18205 - RNA, 20 nt, synthetic construct
  source 1..20: mol_type = other RNA
aaaccctagtctctgtcaag

SEQ ID NO: 18206 - RNA, 20 nt, synthetic construct
  source 1..20: mol_type = other RNA
gagactagggttttagactg

SEQ ID NO: 18207 - RNA, 20 nt, synthetic construct
  source 1..20: mol_type = other RNA
tttagactgaggcttcctgc

SEQ ID NO: 18208 - RNA, 20 nt, synthetic construct
  source 1..20: mol_type = other RNA
ttagactgaggcttcctgca

SEQ ID NO: 18209 - RNA, 20 nt, synthetic construct
  source 1..20: mol_type = other RNA
gggcaatgcgaacaccctgc

SEQ ID NO: 18210 - RNA, 20 nt, synthetic construct
  source 1..20: mol_type = other RNA
gtctgaaggggaacggagaa

SEQ ID NO: 18211 - RNA, 20 nt, synthetic construct
  source 1..20: mol_type = other RNA
ggtctgaaggggaacggaga

SEQ ID NO: 18212 - RNA, 20 nt, synthetic construct
  source 1..20: mol_type = other RNA
cgttccccttcagacctttc

SEQ ID NO: 18213 - RNA, 20 nt, synthetic construct
  source 1..20: mol_type = other RNA
gttccccttcagacctttct

SEQ ID NO: 18214 - RNA, 20 nt, synthetic construct
  source 1..20: mol_type = other RNA
ttccccttcagacctttctg

SEQ ID NO: 18215 - RNA, 20 nt, synthetic construct
  source 1..20: mol_type = other RNA
cagaaaggtctgaaggggaa

SEQ ID NO: 18216 - RNA, 20 nt, synthetic construct
  source 1..20: mol_type = other RNA
ctccccagaaaggtctgaag

SEQ ID NO: 18217 - RNA, 20 nt, synthetic construct
  source 1..20: mol_type = other RNA
tctccccagaaaggtctgaa

SEQ ID NO: 18218 - RNA, 20 nt, synthetic construct
  source 1..20: mol_type = other RNA
ttctccccagaaaggtctga

SEQ ID NO: 18219 - RNA, 20 nt, synthetic construct
  source 1..20: mol_type = other RNA
acctttctggggagaagagg

SEQ ID NO: 18220 - RNA, 20 nt, synthetic construct
  source 1..20: mol_type = other RNA
cctttctggggagaagaggt

SEQ ID NO: 18221 - RNA, 20 nt, synthetic construct
  source 1..20: mol_type = other RNA
ttctggggagaagaggtggg

SEQ ID NO: 18222 - RNA, 20 nt, synthetic construct
  source 1..20: mol_type = other RNA
cccacctcttctccccagaa

SEQ ID NO: 18223 - RNA, 20 nt, synthetic construct
  source 1..20: mol_type = other RNA
tggggagaagaggtgggagg

SEQ ID NO: 18224 - RNA, 20 nt, synthetic construct
  source 1..20: mol_type = other RNA
ggggagaagaggtgggagga

SEQ ID NO: 18225 - RNA, 20 nt, synthetic construct
  source 1..20: mol_type = other RNA
gggagaagaggtgggaggag

SEQ ID NO: 18226 - RNA, 20 nt, synthetic construct
  source 1..20: mol_type = other RNA
gttcatcttattctgaatcc

SEQ ID NO: 18227 - RNA, 20 nt, synthetic construct
  source 1..20: mol_type = other RNA
ctgaatcctggagcagctga

SEQ ID NO: 18228 - RNA, 20 nt, synthetic construct
  source 1..20: mol_type = other RNA
agaaaaccttcagctgctcc

SEQ ID NO: 18229 - RNA, 20 nt, synthetic construct
  source 1..20: mol_type = other RNA
tgaaggttttctcttgagtc

SEQ ID NO: 18230 - RNA, 20 nt, synthetic construct
  source 1..20: mol_type = other RNA
tctcttgagtcaggatgcag

SEQ ID NO: 18231 - RNA, 20 nt, synthetic construct
  source 1..20: mol_type = other RNA
aatgcattaaccagcaagtg

SEQ ID NO: 18232 - RNA, 20 nt, synthetic construct
  source 1..20: mol_type = other RNA
ttaaccagcaagtgtggcca

SEQ ID NO: 18233 - RNA, 20 nt, synthetic construct
  source 1..20: mol_type = other RNA
ttatccttggccacacttgc

SEQ ID NO: 18234 - RNA, 20 nt, synthetic construct
  source 1..20: mol_type = other RNA
ggccaaggataatgaaaaag

SEQ ID NO: 18235 - RNA, 20 nt, synthetic construct
  source 1..20: mol_type = other RNA
gccaaggataatgaaaaagt

SEQ ID NO: 18236 - RNA, 20 nt, synthetic construct
  source 1..20: mol_type = other RNA
ggataatgaaaaagtgggaa

SEQ ID NO: 18237 - RNA, 20 nt, synthetic construct
  source 1..20: mol_type = other RNA
tcccactttttcattatcct

SEQ ID NO: 18238 - RNA, 20 nt, synthetic construct
  source 1..20: mol_type = other RNA
aatgaaaaagtgggaaagga

SEQ ID NO: 18239 - RNA, 20 nt, synthetic construct
  source 1..20: mol_type = other RNA
tgctacaatcagggaggagg

SEQ ID NO: 18240 - RNA, 20 nt, synthetic construct
  source 1..20: mol_type = other RNA
ggatgctacaatcagggagg

SEQ ID NO: 18241 - RNA, 20 nt, synthetic construct
  source 1..20: mol_type = other RNA
gctggatgctacaatcaggg

SEQ ID NO: 18242 - RNA, 20 nt, synthetic construct
  source 1..20: mol_type = other RNA
actgctggatgctacaatca

SEQ ID NO: 18243 - RNA, 20 nt, synthetic construct
  source 1..20: mol_type = other RNA
gactgctggatgctacaatc

SEQ ID NO: 18244 - RNA, 20 nt, synthetic construct
  source 1..20: mol_type = other RNA
atccagcagtctctgtagcc

SEQ ID NO: 18245 - RNA, 20 nt, synthetic construct
  source 1..20: mol_type = other RNA
aacctggctacagagactgc

SEQ ID NO: 18246 - RNA, 20 nt, synthetic construct
  source 1..20: mol_type = other RNA
aatgtggttcttgagtaacc

SEQ ID NO: 18247 - RNA, 20 nt, synthetic construct
  source 1..20: mol_type = other RNA
aagaaccacatttgatttcc

SEQ ID NO: 18248 - RNA, 20 nt, synthetic construct
  source 1..20: mol_type = other RNA
aagggccaggaaatcaaatg

SEQ ID NO: 18249 - RNA, 20 nt, synthetic construct
  source 1..20: mol_type = other RNA
gatttcctggccctttgcct

SEQ ID NO: 18250 - RNA, 20 nt, synthetic construct
  source 1..20: mol_type = other RNA
gccctttgccttggcagtga

SEQ ID NO: 18251 - RNA, 20 nt, synthetic construct
  source 1..20: mol_type = other RNA
cactgccaaggcaaagggcc

SEQ ID NO: 18252 - RNA, 20 nt, synthetic construct
  source 1..20: mol_type = other RNA
gccatcactgccaaggcaaa

SEQ ID NO: 18253 - RNA, 20 nt, synthetic construct
  source 1..20: mol_type = other RNA
tgccatcactgccaaggcaa

SEQ ID NO: 18254 - RNA, 20 nt, synthetic construct
  source 1..20: mol_type = other RNA
taaaaatgccatcactgcca

SEQ ID NO: 18255 - RNA, 20 nt, synthetic construct
  source 1..20: mol_type = other RNA
cttcatttatttttataaca

SEQ ID NO: 18256 - RNA, 20 nt, synthetic construct
  source 1..20: mol_type = other RNA
ttcatttatttttataacat

SEQ ID NO: 18257 - RNA, 20 nt, synthetic construct
  source 1..20: mol_type = other RNA
ttatttttataacatgggtt

SEQ ID NO: 18258 - RNA, 20 nt, synthetic construct
  source 1..20: mol_type = other RNA
tatttttataacatgggtta

SEQ ID NO: 18259 - RNA, 20 nt, synthetic construct
  source 1..20: mol_type = other RNA
tataacatgggttagggaga

SEQ ID NO: 18260 - RNA, 20 nt, synthetic construct
  source 1..20: mol_type = other RNA
ataacatgggttagggagaa

SEQ ID NO: 18261 - RNA, 20 nt, synthetic construct
  source 1..20: mol_type = other RNA
ttagggagaagggccacaaa

SEQ ID NO: 18262 - RNA, 20 nt, synthetic construct
  source 1..20: mol_type = other RNA
gggagaagggccacaaatgg

SEQ ID NO: 18263 - RNA, 20 nt, synthetic construct
  source 1..20: mol_type = other RNA
ggagaagggccacaaatgga

SEQ ID NO: 18264 - RNA, 20 nt, synthetic construct
  source 1..20: mol_type = other RNA
aaggacaatccctccatttg

SEQ ID NO: 18265 - RNA, 20 nt, synthetic construct
  source 1..20: mol_type = other RNA
ctgaagctgtggtgcttgaa

SEQ ID NO: 18266 - RNA, 20 nt, synthetic construct
  source 1..20: mol_type = other RNA
actaattttatctgaagctg

SEQ ID NO: 18267 - RNA, 20 nt, synthetic construct
  source 1..20: mol_type = other RNA
tttaacttaaaaaattctag

SEQ ID NO: 18268 - RNA, 20 nt, synthetic construct
  source 1..20: mol_type = other RNA
ttaacttaaaaaattctaga

SEQ ID NO: 18269 - RNA, 20 nt, synthetic construct
  source 1..20: mol_type = other RNA
aaattctagagggattatat

SEQ ID NO: 18270 - RNA, 20 nt, synthetic construct
  source 1..20: mol_type = other RNA
attggagactcaactgccct

SEQ ID NO: 18271 - RNA, 20 nt, synthetic construct
  source 1..20: mol_type = other RNA
cttggttttagtttataaaa

SEQ ID NO: 18272 - RNA, 20 nt, synthetic construct
  source 1..20: mol_type = other RNA
attttataaactaaaaccaa

SEQ ID NO: 18273 - RNA, 20 nt, synthetic construct
  source 1..20: mol_type = other RNA
cattttataaactaaaacca

SEQ ID NO: 18274 - RNA, 20 nt, synthetic construct
  source 1..20: mol_type = other RNA
tataaaatggcctagtactg

SEQ ID NO: 18275 - RNA, 20 nt, synthetic construct
  source 1..20: mol_type = other RNA
aattaaaattccacagtact

SEQ ID NO: 18276 - RNA, 20 nt, synthetic construct
  source 1..20: mol_type = other RNA
catcccatctgaaacttccc

SEQ ID NO: 18277 - RNA, 20 nt, synthetic construct
  source 1..20: mol_type = other RNA
atcccatctgaaacttccca

SEQ ID NO: 18278 - RNA, 20 nt, synthetic construct
  source 1..20: mol_type = other RNA
tcccatctgaaacttcccag

SEQ ID NO: 18279 - RNA, 20 nt, synthetic construct
  source 1..20: mol_type = other RNA
ctgaaacttcccaggggagt

SEQ ID NO: 18280 - RNA, 20 nt, synthetic construct
  source 1..20: mol_type = other RNA
ctcccctgggaagtttcaga

SEQ ID NO: 18281 - RNA, 20 nt, synthetic construct
  source 1..20: mol_type = other RNA
ctaagaatcccaactcccct

SEQ ID NO: 18282 - RNA, 20 nt, synthetic construct
  source 1..20: mol_type = other RNA
actaagaatcccaactcccc

SEQ ID NO: 18283 - RNA, 20 nt, synthetic construct
  source 1..20: mol_type = other RNA
agttgggattcttagtagat

SEQ ID NO: 18284 - RNA, 20 nt, synthetic construct
  source 1..20: mol_type = other RNA
ttcttagtagattggtagaa

SEQ ID NO: 18285 - RNA, 20 nt, synthetic construct
  source 1..20: mol_type = other RNA
tcttagtagattggtagaaa

SEQ ID NO: 18286 - RNA, 20 nt, synthetic construct
  source 1..20: mol_type = other RNA
cttagtagattggtagaaag

SEQ ID NO: 18287 - RNA, 20 nt, synthetic construct
  source 1..20: mol_type = other RNA
tctactgcatttcccatttt

SEQ ID NO: 18288 - RNA, 20 nt, synthetic construct
  source 1..20: mol_type = other RNA
ctgaacaagataccaaaaat

SEQ ID NO: 18289 - RNA, 20 nt, synthetic construct
  source 1..20: mol_type = other RNA
gctgaacaagataccaaaaa

SEQ ID NO: 18290 - RNA, 20 nt, synthetic construct
  source 1..20: mol_type = other RNA
aagaatgttctcataaatat

SEQ ID NO: 18291 - RNA, 20 nt, synthetic construct
  source 1..20: mol_type = other RNA
ggaaggggtattctatgtgg

SEQ ID NO: 18292 - RNA, 20 nt, synthetic construct
  source 1..20: mol_type = other RNA
ataggaaggggtattctatg

SEQ ID NO: 18293 - RNA, 20 nt, synthetic construct
  source 1..20: mol_type = other RNA
cagagcgagctgataggaag

SEQ ID NO: 18294 - RNA, 20 nt, synthetic construct
  source 1..20: mol_type = other RNA
tcagagcgagctgataggaa

SEQ ID NO: 18295 - RNA, 20 nt, synthetic construct
  source 1..20: mol_type = other RNA
atcagagcgagctgatagga

SEQ ID NO: 18296 - RNA, 20 nt, synthetic construct
  source 1..20: mol_type = other RNA
ctaaatcagagcgagctgat

SEQ ID NO: 18297 - RNA, 20 nt, synthetic construct
  source 1..20: mol_type = other RNA
taaaaaatttaacaaaatta

SEQ ID NO: 18298 - RNA, 20 nt, synthetic construct
  source 1..20: mol_type = other RNA
agatgaatgaagtgctgctg

SEQ ID NO: 18299 - RNA, 20 nt, synthetic construct
  source 1..20: mol_type = other RNA
tcattaaaattacattttta

SEQ ID NO: 18300 - RNA, 20 nt, synthetic construct
  source 1..20: mol_type = other RNA
cctcaaagaaatccaggaaa

SEQ ID NO: 18301 - RNA, 20 nt, synthetic construct
  source 1..20: mol_type = other RNA
aataaaaatgcaaagttcac

SEQ ID NO: 18302 - RNA, 20 nt, synthetic construct
  source 1..20: mol_type = other RNA
tgcatttttattctacatag

SEQ ID NO: 18303 - RNA, 20 nt, synthetic construct
  source 1..20: mol_type = other RNA
tggttctccatgtttttacc

SEQ ID NO: 18304 - RNA, 20 nt, synthetic construct
  source 1..20: mol_type = other RNA
ccatgtttttaccaggaata

SEQ ID NO: 18305 - RNA, 20 nt, synthetic construct
  source 1..20: mol_type = other RNA
ccatattcctggtaaaaaca

SEQ ID NO: 18306 - RNA, 20 nt, synthetic construct
  source 1..20: mol_type = other RNA
caggaatatggtagcatcac

SEQ ID NO: 18307 - RNA, 20 nt, synthetic construct
  source 1..20: mol_type = other RNA
ctgtgatgctaccatattcc

SEQ ID NO: 18308 - RNA, 20 nt, synthetic construct
  source 1..20: mol_type = other RNA
tgcatagatttaaaatgaag

SEQ ID NO: 18309 - RNA, 20 nt, synthetic construct
  source 1..20: mol_type = other RNA
aaaaaatttcacccatcctt

SEQ ID NO: 18310 - RNA, 20 nt, synthetic construct
  source 1..20: mol_type = other RNA
atcaaacatctccaaaggat

SEQ ID NO: 18311 - RNA, 20 nt, synthetic construct
  source 1..20: mol_type = other RNA
tatcaaacatctccaaagga

SEQ ID NO: 18312 - RNA, 20 nt, synthetic construct
  source 1..20: mol_type = other RNA
cttctatcaaacatctccaa

SEQ ID NO: 18313 - RNA, 20 nt, synthetic construct
  source 1..20: mol_type = other RNA
cacagtactaacgaagaggt

SEQ ID NO: 18314 - RNA, 20 nt, synthetic construct
  source 1..20: mol_type = other RNA
acacagtactaacgaagagg

SEQ ID NO: 18315 - RNA, 20 nt, synthetic construct
  source 1..20: mol_type = other RNA
tcgttagtactgtgtgaaat

SEQ ID NO: 18316 - RNA, 20 nt, synthetic construct
  source 1..20: mol_type = other RNA
aattggctgtgatgtgctcg

SEQ ID NO: 18317 - RNA, 20 nt, synthetic construct
  source 1..20: mol_type = other RNA
tgtgatgtgctcgtggttga

SEQ ID NO: 18318 - RNA, 20 nt, synthetic construct
  source 1..20: mol_type = other RNA
gtgatgtgctcgtggttgaa

SEQ ID NO: 18319 - RNA, 20 nt, synthetic construct
  source 1..20: mol_type = other RNA
ggtatgtagtcagcaacccc

SEQ ID NO: 18320 - RNA, 20 nt, synthetic construct
  source 1..20: mol_type = other RNA
tattctctgcttatttccag

SEQ ID NO: 18321 - RNA, 20 nt, synthetic construct
  source 1..20: mol_type = other RNA
ttattctctgcttatttcca

SEQ ID NO: 18322 - RNA, 20 nt, synthetic construct
  source 1..20: mol_type = other RNA
gttattctctgcttatttcc

SEQ ID NO: 18323 - RNA, 20 nt, synthetic construct
  source 1..20: mol_type = other RNA
aataagcagagaataacatg

SEQ ID NO: 18324 - RNA, 20 nt, synthetic construct
  source 1..20: mol_type = other RNA
agaataacatgaggtgactg

SEQ ID NO: 18325 - RNA, 20 nt, synthetic construct
  source 1..20: mol_type = other RNA
gtaaccacctccatccccca

SEQ ID NO: 18326 - RNA, 20 nt, synthetic construct
  source 1..20: mol_type = other RNA
taaccacctccatcccccaa

SEQ ID NO: 18327 - RNA, 20 nt, synthetic construct
  source 1..20: mol_type = other RNA
catcccttgggggatggagg

SEQ ID NO: 18328 - RNA, 20 nt, synthetic construct
  source 1..20: mol_type = other RNA
ctgcatcccttgggggatgg

SEQ ID NO: 18329 - RNA, 20 nt, synthetic construct
  source 1..20: mol_type = other RNA
tcactgcatcccttggggga

SEQ ID NO: 18330 - RNA, 20 nt, synthetic construct
  source 1..20: mol_type = other RNA
tagctcactgcatcccttgg

SEQ ID NO: 18331 - RNA, 20 nt, synthetic construct
  source 1..20: mol_type = other RNA
ctagctcactgcatcccttg

SEQ ID NO: 18332 - RNA, 20 nt, synthetic construct
  source 1..20: mol_type = other RNA
tctagctcactgcatccctt

SEQ ID NO: 18333 - RNA, 20 nt, synthetic construct
  source 1..20: mol_type = other RNA
atctagctcactgcatccct

SEQ ID NO: 18334 - RNA, 20 nt, synthetic construct
  source 1..20: mol_type = other RNA
aacccattaaatgtttttaa

SEQ ID NO: 18335 - RNA, 20 nt, synthetic construct
  source 1..20: mol_type = other RNA
ctcctttaaaaacatttaat

SEQ ID NO: 18336 - RNA, 20 nt, synthetic construct
  source 1..20: mol_type = other RNA
actcctttaaaaacatttaa

SEQ ID NO: 18337 - RNA, 20 nt, synthetic construct
  source 1..20: mol_type = other RNA
agaatgtagccttcagacta

SEQ ID NO: 18338 - RNA, 20 nt, synthetic construct
  source 1..20: mol_type = other RNA
cgttatcttccatagtctga

SEQ ID NO: 18339 - RNA, 20 nt, synthetic construct
  source 1..20: mol_type = other RNA
ggtgagggaagaaaagacat

SEQ ID NO: 18340 - RNA, 20 nt, synthetic construct
  source 1..20: mol_type = other RNA
cttccctcaccttcattcaa

SEQ ID NO: 18341 - RNA, 20 nt, synthetic construct
  source 1..20: mol_type = other RNA
acacctttgaatgaaggtga

SEQ ID NO: 18342 - RNA, 20 nt, synthetic construct
  source 1..20: mol_type = other RNA
aacacctttgaatgaaggtg

SEQ ID NO: 18343 - RNA, 20 nt, synthetic construct
  source 1..20: mol_type = other RNA
ggtgtaacacctttgaatga

SEQ ID NO: 18344 - RNA, 20 nt, synthetic construct
  source 1..20: mol_type = other RNA
acatactggcagtttcttag

SEQ ID NO: 18345 - RNA, 20 nt, synthetic construct
  source 1..20: mol_type = other RNA
atgttaatcacaagacatac

SEQ ID NO: 18346 - RNA, 20 nt, synthetic construct
  source 1..20: mol_type = other RNA
ctcttctatcaacaatatcg

SEQ ID NO: 18347 - RNA, 20 nt, synthetic construct
  source 1..20: mol_type = other RNA
tgttgatagaagagacgaca

SEQ ID NO: 18348 - RNA, 20 nt, synthetic construct
  source 1..20: mol_type = other RNA
aaggccccaagatgtcattg

SEQ ID NO: 18349 - RNA, 20 nt, synthetic construct
  source 1..20: mol_type = other RNA
gaaaccacaatgacatcttg

SEQ ID NO: 18350 - RNA, 20 nt, synthetic construct
  source 1..20: mol_type = other RNA
tgaaaccacaatgacatctt

SEQ ID NO: 18351 - RNA, 20 nt, synthetic construct
  source 1..20: mol_type = other RNA
ttgaaaccacaatgacatct

SEQ ID NO: 18352 - RNA, 20 nt, synthetic construct
  source 1..20: mol_type = other RNA
tatgattaacatctcacttt

SEQ ID NO: 18353 - RNA, 20 nt, synthetic construct
  source 1..20: mol_type = other RNA
ttaacatctcactttaggtc

SEQ ID NO: 18354 - RNA, 20 nt, synthetic construct
  source 1..20: mol_type = other RNA
taacatctcactttaggtca

SEQ ID NO: 18355 - RNA, 20 nt, synthetic construct
  source 1..20: mol_type = other RNA
actttaggtcagggaataag

SEQ ID NO: 18356 - RNA, 20 nt, synthetic construct
  source 1..20: mol_type = other RNA
gggaataagcggtaagatga

SEQ ID NO: 18357 - RNA, 20 nt, synthetic construct
  source 1..20: mol_type = other RNA
ggaataagcggtaagatgaa

SEQ ID NO: 18358 - RNA, 20 nt, synthetic construct
  source 1..20: mol_type = other RNA
taattaattttttagagaca

SEQ ID NO: 18359 - RNA, 20 nt, synthetic construct
  source 1..20: mol_type = other RNA
aataaaaatctgttatcaaa

SEQ ID NO: 18360 - RNA, 20 nt, synthetic construct
  source 1..20: mol_type = other RNA
ttatcaaaaggaaaaaaatt

SEQ ID NO: 18361 - RNA, 20 nt, synthetic construct
  source 1..20: mol_type = other RNA
aggaaaaaaattaggaaaac

SEQ ID NO: 18362 - RNA, 20 nt, synthetic construct
  source 1..20: mol_type = other RNA
aaaaaattaggaaaacagga

SEQ ID NO: 18363 - RNA, 20 nt, synthetic construct
  source 1..20: mol_type = other RNA
aaaacaggatggataaaaaa

SEQ ID NO: 18364 - RNA, 20 nt, synthetic construct
  source 1..20: mol_type = other RNA
aaacaggatggataaaaaat

SEQ ID NO: 18365 - RNA, 20 nt, synthetic construct
  source 1..20: mol_type = other RNA
aaaaaatgggaattcagatc

SEQ ID NO: 18366 - RNA, 20 nt, synthetic construct
  source 1..20: mol_type = other RNA
tgtcattcatcattctctca

SEQ ID NO: 18367 - RNA, 20 nt, synthetic construct
  source 1..20: mol_type = other RNA
tgtaatactcacttgaacat

SEQ ID NO: 18368 - RNA, 20 nt, synthetic construct
  source 1..20: mol_type = other RNA
ttttgcgctgtgcttcctct

SEQ ID NO: 18369 - RNA, 20 nt, synthetic construct
  source 1..20: mol_type = other RNA
agtgttacttgttgtcctag

SEQ ID NO: 18370 - RNA, 20 nt, synthetic construct
  source 1..20: mol_type = other RNA
acttttcacactaacattga

SEQ ID NO: 18371 - RNA, 20 nt, synthetic construct
  source 1..20: mol_type = other RNA
tcaatgttagtgtgaaaagt

SEQ ID NO: 18372 - RNA, 20 nt, synthetic construct
  source 1..20: mol_type = other RNA
atcaatgttagtgtgaaaag

SEQ ID NO: 18373 - RNA, 20 nt, synthetic construct
  source 1..20: mol_type = other RNA
gcagctcaacccccctcagc

SEQ ID NO: 18374 - RNA, 20 nt, synthetic construct
  source 1..20: mol_type = other RNA
ccccctcagctggttattta

SEQ ID NO: 18375 - RNA, 20 nt, synthetic construct
  source 1..20: mol_type = other RNA
cataaataaccagctgaggg

SEQ ID NO: 18376 - RNA, 20 nt, synthetic construct
  source 1..20: mol_type = other RNA
ccataaataaccagctgagg

SEQ ID NO: 18377 - RNA, 20 nt, synthetic construct
  source 1..20: mol_type = other RNA
accataaataaccagctgag

SEQ ID NO: 18378 - RNA, 20 nt, synthetic construct
  source 1..20: mol_type = other RNA
caccataaataaccagctga

SEQ ID NO: 18379 - RNA, 20 nt, synthetic construct
  source 1..20: mol_type = other RNA
acaccataaataaccagctg

SEQ ID NO: 18380 - RNA, 20 nt, synthetic construct
  source 1..20: mol_type = other RNA
gacagtgatgttagatgcag

SEQ ID NO: 18381 - RNA, 20 nt, synthetic construct
  source 1..20: mol_type = other RNA
agtgatgttagatgcagagg

SEQ ID NO: 18382 - RNA, 20 nt, synthetic construct
  source 1..20: mol_type = other RNA
gtgatgttagatgcagaggt

SEQ ID NO: 18383 - RNA, 20 nt, synthetic construct
  source 1..20: mol_type = other RNA
tgatgttagatgcagaggtg

SEQ ID NO: 18384 - RNA, 20 nt, synthetic construct
  source 1..20: mol_type = other RNA
ttagatgcagaggtggggcc

SEQ ID NO: 18385 - RNA, 20 nt, synthetic construct
  source 1..20: mol_type = other RNA
tagatgcagaggtggggcca

SEQ ID NO: 18386 - RNA, 20 nt, synthetic construct
  source 1..20: mol_type = other RNA
gcagaggtggggccagggcc

SEQ ID NO: 18387 - RNA, 20 nt, synthetic construct
  source 1..20: mol_type = other RNA
cagaggtggggccagggcca

SEQ ID NO: 18388 - RNA, 20 nt, synthetic construct
  source 1..20: mol_type = other RNA
ggggccagggccagggttgc

SEQ ID NO: 18389 - RNA, 20 nt, synthetic construct
  source 1..20: mol_type = other RNA
gggccagggccagggttgct

SEQ ID NO: 18390 - RNA, 20 nt, synthetic construct
  source 1..20: mol_type = other RNA
ctacccagcaaccctggccc

SEQ ID NO: 18391 - RNA, 20 nt, synthetic construct
  source 1..20: mol_type = other RNA
ccagggttgctgggtagagt

SEQ ID NO: 18392 - RNA, 20 nt, synthetic construct
  source 1..20: mol_type = other RNA
ccaactctacccagcaaccc

SEQ ID NO: 18393 - RNA, 20 nt, synthetic construct
  source 1..20: mol_type = other RNA
ttgtacctcatgatctgtga

SEQ ID NO: 18394 - RNA, 20 nt, synthetic construct
  source 1..20: mol_type = other RNA
tgtacctcatgatctgtgaa

SEQ ID NO: 18395 - RNA, 20 nt, synthetic construct
  source 1..20: mol_type = other RNA
atgatctgtgaagggcaaag

SEQ ID NO: 18396 - RNA, 20 nt, synthetic construct
  source 1..20: mol_type = other RNA
tttgcccttcacagatcatg

SEQ ID NO: 18397 - RNA, 20 nt, synthetic construct
  source 1..20: mol_type = other RNA
gccacatttgtcaaagatta

SEQ ID NO: 18398 - RNA, 20 nt, synthetic construct
  source 1..20: mol_type = other RNA
ccacatttgtcaaagattat

SEQ ID NO: 18399 - RNA, 20 nt, synthetic construct
  source 1..20: mol_type = other RNA
cacatttgtcaaagattatg

SEQ ID NO: 18400 - RNA, 20 nt, synthetic construct
  source 1..20: mol_type = other RNA
cccataatctttgacaaatg

SEQ ID NO: 18401 - RNA, 20 nt, synthetic construct
  source 1..20: mol_type = other RNA
gattatggggtttgtatcat

SEQ ID NO: 18402 - RNA, 20 nt, synthetic construct
  source 1..20: mol_type = other RNA
aggtgcaaaatctctgttat

SEQ ID NO: 18403 - RNA, 20 nt, synthetic construct
  source 1..20: mol_type = other RNA
ctttctcaaaatgtcttctg

SEQ ID NO: 18404 - RNA, 20 nt, synthetic construct
  source 1..20: mol_type = other RNA
actttctcaaaatgtcttct

SEQ ID NO: 18405 - RNA, 20 nt, synthetic construct
  source 1..20: mol_type = other RNA
tactttctcaaaatgtcttc

SEQ ID NO: 18406 - RNA, 20 nt, synthetic construct
  source 1..20: mol_type = other RNA
ctctgcccacatgggaataa

SEQ ID NO: 18407 - RNA, 20 nt, synthetic construct
  source 1..20: mol_type = other RNA
aatgtccattattcccatgt

SEQ ID NO: 18408 - RNA, 20 nt, synthetic construct
  source 1..20: mol_type = other RNA
taatgtccattattcccatg

SEQ ID NO: 18409 - RNA, 20 nt, synthetic construct
  source 1..20: mol_type = other RNA
atcaatgttaagtggcatat

SEQ ID NO: 18410 - RNA, 20 nt, synthetic construct
  source 1..20: mol_type = other RNA
acatgtggatcaatgttaag

SEQ ID NO: 18411 - RNA, 20 nt, synthetic construct
  source 1..20: mol_type = other RNA
attgatccacatgtcatttc

SEQ ID NO: 18412 - RNA, 20 nt, synthetic construct
  source 1..20: mol_type = other RNA
cttatgccagaaatgacatg

SEQ ID NO: 18413 - RNA, 20 nt, synthetic construct
  source 1..20: mol_type = other RNA
agttgctgctttatgacata

SEQ ID NO: 18414 - RNA, 20 nt, synthetic construct
  source 1..20: mol_type = other RNA
ctgctttatgacataaggag

SEQ ID NO: 18415 - RNA, 20 nt, synthetic construct
  source 1..20: mol_type = other RNA
ctttatgacataaggagagg

SEQ ID NO: 18416 - RNA, 20 nt, synthetic construct
  source 1..20: mol_type = other RNA
ggagaggtggatgtcttacc

SEQ ID NO: 18417 - RNA, 20 nt, synthetic construct
  source 1..20: mol_type = other RNA
taccaggactacaagtgacc

SEQ ID NO: 18418 - RNA, 20 nt, synthetic construct
  source 1..20: mol_type = other RNA
accaggactacaagtgacct

SEQ ID NO: 18419 - RNA, 20 nt, synthetic construct
  source 1..20: mol_type = other RNA
ccaggactacaagtgacctg

SEQ ID NO: 18420 - RNA, 20 nt, synthetic construct
  source 1..20: mol_type = other RNA
ccccaggtcacttgtagtcc

SEQ ID NO: 18421 - RNA, 20 nt, synthetic construct
  source 1..20: mol_type = other RNA
aagtgacctggggcacatct

SEQ ID NO: 18422 - RNA, 20 nt, synthetic construct
  source 1..20: mol_type = other RNA
gacatacctagatgtgcccc

SEQ ID NO: 18423 - RNA, 20 nt, synthetic construct
  source 1..20: mol_type = other RNA
ctaggtatgtcttgcctttc

SEQ ID NO: 18424 - RNA, 20 nt, synthetic construct
  source 1..20: mol_type = other RNA
taggtatgtcttgcctttca

SEQ ID NO: 18425 - RNA, 20 nt, synthetic construct
  source 1..20: mol_type = other RNA
tatgtcttgcctttcaggga

SEQ ID NO: 18426 - RNA, 20 nt, synthetic construct
  source 1..20: mol_type = other RNA
atgtcttgcctttcagggaa

SEQ ID NO: 18427 - RNA, 20 nt, synthetic construct
  source 1..20: mol_type = other RNA
tcttgcctttcagggaaggg

SEQ ID NO: 18428 - RNA, 20 nt, synthetic construct
  source 1..20: mol_type = other RNA
caaatcctcccttccctgaa

SEQ ID NO: 18429 - RNA, 20 nt, synthetic construct
  source 1..20: mol_type = other RNA
ggaagggaggatttgagcaa

SEQ ID NO: 18430 - RNA, 20 nt, synthetic construct
  source 1..20: mol_type = other RNA
gaggatttgagcaatggaca

SEQ ID NO: 18431 - RNA, 20 nt, synthetic construct
  source 1..20: mol_type = other RNA
aggatttgagcaatggacat

SEQ ID NO: 18432 - RNA, 20 nt, synthetic construct
  source 1..20: mol_type = other RNA
ggatttgagcaatggacatg

SEQ ID NO: 18433 - RNA, 20 nt, synthetic construct
  source 1..20: mol_type = other RNA
gagcaatggacatggggttg

SEQ ID NO: 18434 - RNA, 20 nt, synthetic construct
  source 1..20: mol_type = other RNA
tactcaatgagattaagcag

SEQ ID NO: 18435 - RNA, 20 nt, synthetic construct
  source 1..20: mol_type = other RNA
atactcaatgagattaagca

SEQ ID NO: 18436 - RNA, 20 nt, synthetic construct
  source 1..20: mol_type = other RNA
gatactcaatgagattaagc

SEQ ID NO: 18437 - RNA, 20 nt, synthetic construct
  source 1..20: mol_type = other RNA
atggaactgcaagaagacta

SEQ ID NO: 18438 - RNA, 20 nt, synthetic construct
  source 1..20: mol_type = other RNA
cagttccattcctttttaga

SEQ ID NO: 18439 - RNA, 20 nt, synthetic construct
  source 1..20: mol_type = other RNA
cattcctttttagatggctc

SEQ ID NO: 18440 - RNA, 20 nt, synthetic construct
  source 1..20: mol_type = other RNA
ctgagccatctaaaaaggaa

SEQ ID NO: 18441 - RNA, 20 nt, synthetic construct
  source 1..20: mol_type = other RNA
aacacctgagccatctaaaa

SEQ ID NO: 18442 - RNA, 20 nt, synthetic construct
  source 1..20: mol_type = other RNA
caggtgttacagagagagcc

SEQ ID NO: 18443 - RNA, 20 nt, synthetic construct
  source 1..20: mol_type = other RNA
aggtgttacagagagagcct

SEQ ID NO: 18444 - RNA, 20 nt, synthetic construct
  source 1..20: mol_type = other RNA
gttacagagagagcctggga

SEQ ID NO: 18445 - RNA, 20 nt, synthetic construct
  source 1..20: mol_type = other RNA
ctctttctgtcttccttccc

SEQ ID NO: 18446 - RNA, 20 nt, synthetic construct
  source 1..20: mol_type = other RNA
aagagagagaaagagtaatt

SEQ ID NO: 18447 - RNA, 20 nt, synthetic construct
  source 1..20: mol_type = other RNA
aattaggcatagctgagagt

SEQ ID NO: 18448 - RNA, 20 nt, synthetic construct
  source 1..20: mol_type = other RNA
ataaacttgatcactaatca

SEQ ID NO: 18449 - RNA, 20 nt, synthetic construct
  source 1..20: mol_type = other RNA
atatctcaggtcatactagc

SEQ ID NO: 18450 - RNA, 20 nt, synthetic construct
  source 1..20: mol_type = other RNA
cagagatgttagtagaagcc

SEQ ID NO: 18451 - RNA, 20 nt, synthetic construct
  source 1..20: mol_type = other RNA
gcctcttgattctgcaatcc

SEQ ID NO: 18452 - RNA, 20 nt, synthetic construct
  source 1..20: mol_type = other RNA
gattgcagaatcaagaggcc

SEQ ID NO: 18453 - RNA, 20 nt, synthetic construct
  source 1..20: mol_type = other RNA
gcctggattgcagaatcaag

SEQ ID NO: 18454 - RNA, 20 nt, synthetic construct
  source 1..20: mol_type = other RNA
attctgcaatccaggcttat

SEQ ID NO: 18455 - RNA, 20 nt, synthetic construct
  source 1..20: mol_type = other RNA
tgcaatccaggcttattggc

SEQ ID NO: 18456 - RNA, 20 nt, synthetic construct
  source 1..20: mol_type = other RNA
tgggttcctgccaataagcc

SEQ ID NO: 18457 - RNA, 20 nt, synthetic construct
  source 1..20: mol_type = other RNA
cgtgctggatgctcttggtt

SEQ ID NO: 18458 - RNA, 20 nt, synthetic construct
  source 1..20: mol_type = other RNA
acgtgctggatgctcttggt

SEQ ID NO: 18459 - RNA, 20 nt, synthetic construct
  source 1..20: mol_type = other RNA
aaacacgtgctggatgctct

SEQ ID NO: 18460 - RNA, 20 nt, synthetic construct
  source 1..20: mol_type = other RNA
ccagcacgtgtttacctgca

SEQ ID NO: 18461 - RNA, 20 nt, synthetic construct
  source 1..20: mol_type = other RNA
acgtgtttacctgcatggcg

SEQ ID NO: 18462 - RNA, 20 nt, synthetic construct
  source 1..20: mol_type = other RNA
cagtactggcctcgccatgc

SEQ ID NO: 18463 - RNA, 20 nt, synthetic construct
  source 1..20: mol_type = other RNA
attggagacatctacagtac

SEQ ID NO: 18464 - RNA, 20 nt, synthetic construct
  source 1..20: mol_type = other RNA
atcaaagataatggcatcat

SEQ ID NO: 18465 - RNA, 20 nt, synthetic construct
  source 1..20: mol_type = other RNA
agcatgaagatcaaagataa

SEQ ID NO: 18466 - RNA, 20 nt, synthetic construct
  source 1..20: mol_type = other RNA
tcaggtactaaaggatattg

SEQ ID NO: 18467 - RNA, 20 nt, synthetic construct
  source 1..20: mol_type = other RNA
cctttagtacctgaccaaac

SEQ ID NO: 18468 - RNA, 20 nt, synthetic construct
  source 1..20: mol_type = other RNA
ctttagtacctgaccaaaca

SEQ ID NO: 18469 - RNA, 20 nt, synthetic construct
  source 1..20: mol_type = other RNA
cctgtttggtcaggtactaa

SEQ ID NO: 18470 - RNA, 20 nt, synthetic construct
  source 1..20: mol_type = other RNA
ttacagatccctgtttggtc

SEQ ID NO: 18471 - RNA, 20 nt, synthetic construct
  source 1..20: mol_type = other RNA
gaaggttacagatccctgtt

SEQ ID NO: 18472 - RNA, 20 nt, synthetic construct
  source 1..20: mol_type = other RNA
taaccttcctctgaacctac

SEQ ID NO: 18473 - RNA, 20 nt, synthetic construct
  source 1..20: mol_type = other RNA
aaccttcctctgaacctaca

SEQ ID NO: 18474 - RNA, 20 nt, synthetic construct
  source 1..20: mol_type = other RNA
atccctgtaggttcagagga

SEQ ID NO: 18475 - RNA, 20 nt, synthetic construct
  source 1..20: mol_type = other RNA
caagatccctgtaggttcag

SEQ ID NO: 18476 - RNA, 20 nt, synthetic construct
  source 1..20: mol_type = other RNA
atgtacaacaagatccctgt

SEQ ID NO: 18477 - RNA, 20 nt, synthetic construct
  source 1..20: mol_type = other RNA
gtacatacaggtcagagcca

SEQ ID NO: 18478 - RNA, 20 nt, synthetic construct
  source 1..20: mol_type = other RNA
cacaggagcaatggcaacct

SEQ ID NO: 18479 - RNA, 20 nt, synthetic construct
  source 1..20: mol_type = other RNA
attcacagacacaggagcaa

SEQ ID NO: 18480 - RNA, 20 nt, synthetic construct
  source 1..20: mol_type = other RNA
cctgtgtctgtgaatgacag

SEQ ID NO: 18481 - RNA, 20 nt, synthetic construct
  source 1..20: mol_type = other RNA
ctgtgtctgtgaatgacaga

SEQ ID NO: 18482 - RNA, 20 nt, synthetic construct
  source 1..20: mol_type = other RNA
cctctgtcattcacagacac

SEQ ID NO: 18483 - RNA, 20 nt, synthetic construct
  source 1..20: mol_type = other RNA
tattgctgtgatggtgacta

SEQ ID NO: 18484 - RNA, 20 nt, synthetic construct
  source 1..20: mol_type = other RNA
agctgttcatattgctgtga

SEQ ID NO: 18485 - RNA, 20 nt, synthetic construct
  source 1..20: mol_type = other RNA
attgtgtgcttattatattc

SEQ ID NO: 18486 - RNA, 20 nt, synthetic construct
  source 1..20: mol_type = other RNA
ctgaggagcaaataaaatca

SEQ ID NO: 18487 - RNA, 20 nt, synthetic construct
  source 1..20: mol_type = other RNA
catccttagctcctcctcca

SEQ ID NO: 18488 - RNA, 20 nt, synthetic construct
  source 1..20: mol_type = other RNA
atccttagctcctcctccat

SEQ ID NO: 18489 - RNA, 20 nt, synthetic construct
  source 1..20: mol_type = other RNA
gtcccatggaggaggagcta

SEQ ID NO: 18490 - RNA, 20 nt, synthetic construct
  source 1..20: mol_type = other RNA
aggagagcgtcccatggagg

SEQ ID NO: 18491 - RNA, 20 nt, synthetic construct
  source 1..20: mol_type = other RNA
caaaggagagcgtcccatgg

SEQ ID NO: 18492 - RNA, 20 nt, synthetic construct
  source 1..20: mol_type = other RNA
tgacaaaggagagcgtccca

SEQ ID NO: 18493 - RNA, 20 nt, synthetic construct
  source 1..20: mol_type = other RNA
agctggcagggaagtgacaa

SEQ ID NO: 18494 - RNA, 20 nt, synthetic construct
  source 1..20: mol_type = other RNA
actgaatggtggagctggca

SEQ ID NO: 18495 - RNA, 20 nt, synthetic construct
  source 1..20: mol_type = other RNA
aactgaatggtggagctggc

SEQ ID NO: 18496 - RNA, 20 nt, synthetic construct
  source 1..20: mol_type = other RNA
cgtgaactgaatggtggagc

SEQ ID NO: 18497 - RNA, 20 nt, synthetic construct
  source 1..20: mol_type = other RNA
aggcatcgtgaactgaatgg

SEQ ID NO: 18498 - RNA, 20 nt, synthetic construct
  source 1..20: mol_type = other RNA
cagaggcatcgtgaactgaa

SEQ ID NO: 18499 - RNA, 20 nt, synthetic construct
  source 1..20: mol_type = other RNA
tgcctctgatgttcccagct

SEQ ID NO: 18500 - RNA, 20 nt, synthetic construct
  source 1..20: mol_type = other RNA
gcctctgatgttcccagctc

SEQ ID NO: 18501 - RNA, 20 nt, synthetic construct
  source 1..20: mol_type = other RNA
cctctgatgttcccagctcg

SEQ ID NO: 18502 - RNA, 20 nt, synthetic construct
  source 1..20: mol_type = other RNA
ccccgagctgggaacatcag

SEQ ID NO: 18503 - RNA, 20 nt, synthetic construct
  source 1..20: mol_type = other RNA
atgttcccagctcggggtag

SEQ ID NO: 18504 - RNA, 20 nt, synthetic construct
  source 1..20: mol_type = other RNA
ggtcaccactaccccgagct

SEQ ID NO: 18505 - RNA, 20 nt, synthetic construct
  source 1..20: mol_type = other RNA
aggtcaccactaccccgagc

SEQ ID NO: 18506 - RNA, 20 nt, synthetic construct
  source 1..20: mol_type = other RNA
gacctactcacctacattga

SEQ ID NO: 18507 - RNA, 20 nt, synthetic construct
  source 1..20: mol_type = other RNA
acctactcacctacattgaa

SEQ ID NO: 18508 - RNA, 20 nt, synthetic construct
  source 1..20: mol_type = other RNA
ctcacctacattgaagggag

SEQ ID NO: 18509 - RNA, 20 nt, synthetic construct
  source 1..20: mol_type = other RNA
tcccttcaatgtaggtgagt

SEQ ID NO: 18510 - RNA, 20 nt, synthetic construct
  source 1..20: mol_type = other RNA
tacattgaagggagaggagt

SEQ ID NO: 18511 - RNA, 20 nt, synthetic construct
  source 1..20: mol_type = other RNA
aactcctctcccttcaatgt

SEQ ID NO: 18512 - RNA, 20 nt, synthetic construct
  source 1..20: mol_type = other RNA
agggagaggagttggccagc

SEQ ID NO: 18513 - RNA, 20 nt, synthetic construct
  source 1..20: mol_type = other RNA
gggagaggagttggccagca

SEQ ID NO: 18514 - RNA, 20 nt, synthetic construct
  source 1..20: mol_type = other RNA
ggagttggccagcagggtct

SEQ ID NO: 18515 - RNA, 20 nt, synthetic construct
  source 1..20: mol_type = other RNA
ccagcagggtcttggcaaag

SEQ ID NO: 18516 - RNA, 20 nt, synthetic construct
  source 1..20: mol_type = other RNA
cagggtcttggcaaagcgga

SEQ ID NO: 18517 - RNA, 20 nt, synthetic construct
  source 1..20: mol_type = other RNA
ccgctttgccaagaccctgc

SEQ ID NO: 18518 - RNA, 20 nt, synthetic construct
  source 1..20: mol_type = other RNA
ttggcaaagcggacggctat

SEQ ID NO: 18519 - RNA, 20 nt, synthetic construct
  source 1..20: mol_type = other RNA
aaagcggacggctatcggca

SEQ ID NO: 18520 - RNA, 20 nt, synthetic construct
  source 1..20: mol_type = other RNA
aggtcgcctcagagttcttc

SEQ ID NO: 18521 - RNA, 20 nt, synthetic construct
  source 1..20: mol_type = other RNA
actgtgccagaagaactctg

SEQ ID NO: 18522 - RNA, 20 nt, synthetic construct
  source 1..20: mol_type = other RNA
cagtgccaagatcgctagac

SEQ ID NO: 18523 - RNA, 20 nt, synthetic construct
  source 1..20: mol_type = other RNA
agtgccaagatcgctagact

SEQ ID NO: 18524 - RNA, 20 nt, synthetic construct
  source 1..20: mol_type = other RNA
tgggcccagtctagcgatct

SEQ ID NO: 18525 - RNA, 20 nt, synthetic construct
  source 1..20: mol_type = other RNA
cgctagactgggcccataga

SEQ ID NO: 18526 - RNA, 20 nt, synthetic construct
  source 1..20: mol_type = other RNA
ctgaagcatcagccttctat

SEQ ID NO: 18527 - RNA, 20 nt, synthetic construct
  source 1..20: mol_type = other RNA
gctgaagcatcagccttcta

SEQ ID NO: 18528 - RNA, 20 nt, synthetic construct
  source 1..20: mol_type = other RNA
aaggctgatgcttcagcgtt

SEQ ID NO: 18529 - RNA, 20 nt, synthetic construct
  source 1..20: mol_type = other RNA
aggctgatgcttcagcgttg

SEQ ID NO: 18530 - RNA, 20 nt, synthetic construct
  source 1..20: mol_type = other RNA
ttcagcgttggggcctccga

SEQ ID NO: 18531 - RNA, 20 nt, synthetic construct
  source 1..20: mol_type = other RNA
tcagcgttggggcctccgaa

SEQ ID NO: 18532 - RNA, 20 nt, synthetic construct
  source 1..20: mol_type = other RNA
cagcgttggggcctccgaag

SEQ ID NO: 18533 - RNA, 20 nt, synthetic construct
  source 1..20: mol_type = other RNA
aggttctctatccccttcgg

SEQ ID NO: 18534 - RNA, 20 nt, synthetic construct
  source 1..20: mol_type = other RNA
tgaaggttctctatcccctt

SEQ ID NO: 18535 - RNA, 20 nt, synthetic construct
  source 1..20: mol_type = other RNA
ggtgactgtgagtctgatga

SEQ ID NO: 18536 - RNA, 20 nt, synthetic construct
  source 1..20: mol_type = other RNA
gactcacagtcaccacgatg

SEQ ID NO: 18537 - RNA, 20 nt, synthetic construct
  source 1..20: mol_type = other RNA
gatgaggacatttgcaaaga

SEQ ID NO: 18538 - RNA, 20 nt, synthetic construct
  source 1..20: mol_type = other RNA
ctttgcaaatgtcctcatcg

SEQ ID NO: 18539 - RNA, 20 nt, synthetic construct
  source 1..20: mol_type = other RNA
gaaaagccaagcctttgaaa

SEQ ID NO: 18540 - RNA, 20 nt, synthetic construct
  source 1..20: mol_type = other RNA
caatttccttttcaaaggct

SEQ ID NO: 18541 - RNA, 20 nt, synthetic construct
  source 1..20: mol_type = other RNA
tctagcaatttccttttcaa

SEQ ID NO: 18542 - RNA, 20 nt, synthetic construct
  source 1..20: mol_type = other RNA
gtggagagaaaggcaagtta

SEQ ID NO: 18543 - RNA, 20 nt, synthetic construct
  source 1..20: mol_type = other RNA
ggtggagagaaaggcaagtt

SEQ ID NO: 18544 - RNA, 20 nt, synthetic construct
  source 1..20: mol_type = other RNA
aagggtgggggtggagagaa

SEQ ID NO: 18545 - RNA, 20 nt, synthetic construct
  source 1..20: mol_type = other RNA
acccccacccttttcctttc

SEQ ID NO: 18546 - RNA, 20 nt, synthetic construct
  source 1..20: mol_type = other RNA
cccccacccttttcctttct

SEQ ID NO: 18547 - RNA, 20 nt, synthetic construct
  source 1..20: mol_type = other RNA
agaaaggaaaagggtggggg

SEQ ID NO: 18548 - RNA, 20 nt, synthetic construct
  source 1..20: mol_type = other RNA
cccagaaaggaaaagggtgg

SEQ ID NO: 18549 - RNA, 20 nt, synthetic construct
  source 1..20: mol_type = other RNA
acccagaaaggaaaagggtg

SEQ ID NO: 18550 - RNA, 20 nt, synthetic construct
  source 1..20: mol_type = other RNA
aacccagaaaggaaaagggt

SEQ ID NO: 18551 - RNA, 20 nt, synthetic construct
  source 1..20: mol_type = other RNA
aaacccagaaaggaaaaggg

SEQ ID NO: 18552 - RNA, 20 nt, synthetic construct
  source 1..20: mol_type = other RNA
tttaaacccagaaaggaaaa

SEQ ID NO: 18553 - RNA, 20 nt, synthetic construct
  source 1..20: mol_type = other RNA
ttttaaacccagaaaggaaa

SEQ ID NO: 18554 - RNA, 20 nt, synthetic construct
  source 1..20: mol_type = other RNA
tttctgggtttaaaattctt

SEQ ID NO: 18555 - RNA, 20 nt, synthetic construct
  source 1..20: mol_type = other RNA
taagaattttaaacccagaa

SEQ ID NO: 18556 - RNA, 20 nt, synthetic construct
  source 1..20: mol_type = other RNA
ggagaaaagagtcaggcata

SEQ ID NO: 18557 - RNA, 20 nt, synthetic construct
  source 1..20: mol_type = other RNA
ctggaagggagaaaagagtc

SEQ ID NO: 18558 - RNA, 20 nt, synthetic construct
  source 1..20: mol_type = other RNA
cccttccagtcaggtcttac

SEQ ID NO: 18559 - RNA, 20 nt, synthetic construct
  source 1..20: mol_type = other RNA
tccagtcaggtcttactgga

SEQ ID NO: 18560 - RNA, 20 nt, synthetic construct
  source 1..20: mol_type = other RNA
ccagtaagacctgactggaa

SEQ ID NO: 18561 - RNA, 20 nt, synthetic construct
  source 1..20: mol_type = other RNA
tccagtaagacctgactgga

SEQ ID NO: 18562 - RNA, 20 nt, synthetic construct
  source 1..20: mol_type = other RNA
accttccagtaagacctgac

SEQ ID NO: 18563 - RNA, 20 nt, synthetic construct
  source 1..20: mol_type = other RNA
acaaagacaaatggagaact

SEQ ID NO: 18564 - RNA, 20 nt, synthetic construct
  source 1..20: mol_type = other RNA
tacaaagacaaatggagaac

SEQ ID NO: 18565 - RNA, 20 nt, synthetic construct
  source 1..20: mol_type = other RNA
ctccatttgtctttgtagaa

SEQ ID NO: 18566 - RNA, 20 nt, synthetic construct
  source 1..20: mol_type = other RNA
atccattctacaaagacaaa

SEQ ID NO: 18567 - RNA, 20 nt, synthetic construct
  source 1..20: mol_type = other RNA
agaatggatactttatcccc

SEQ ID NO: 18568 - RNA, 20 nt, synthetic construct
  source 1..20: mol_type = other RNA
gaatggatactttatcccca

SEQ ID NO: 18569 - RNA, 20 nt, synthetic construct
  source 1..20: mol_type = other RNA
atactttatccccagggtct

SEQ ID NO: 18570 - RNA, 20 nt, synthetic construct
  source 1..20: mol_type = other RNA
tttatccccagggtctcggc

SEQ ID NO: 18571 - RNA, 20 nt, synthetic construct
  source 1..20: mol_type = other RNA
atccccagggtctcggcagg

SEQ ID NO: 18572 - RNA, 20 nt, synthetic construct
  source 1..20: mol_type = other RNA
cccagggtctcggcaggagg

SEQ ID NO: 18573 - RNA, 20 nt, synthetic construct
  source 1..20: mol_type = other RNA
ctcctcctgccgagaccctg

SEQ ID NO: 18574 - RNA, 20 nt, synthetic construct
  source 1..20: mol_type = other RNA
cctcctcctgccgagaccct

SEQ ID NO: 18575 - RNA, 20 nt, synthetic construct
  source 1..20: mol_type = other RNA
gtctcggcaggaggaggtga

SEQ ID NO: 18576 - RNA, 20 nt, synthetic construct
  source 1..20: mol_type = other RNA
ggaggaggtgagggccatga

SEQ ID NO: 18577 - RNA, 20 nt, synthetic construct
  source 1..20: mol_type = other RNA
aggtgagggccatgatggtg

SEQ ID NO: 18578 - RNA, 20 nt, synthetic construct
  source 1..20: mol_type = other RNA
gcagctcggcctcaccatca

SEQ ID NO: 18579 - RNA, 20 nt, synthetic construct
  source 1..20: mol_type = other RNA
ggtgaggccgagctgcccaa

SEQ ID NO: 18580 - RNA, 20 nt, synthetic construct
  source 1..20: mol_type = other RNA
gatctaaccattgggcagct

SEQ ID NO: 18581 - RNA, 20 nt, synthetic construct
  source 1..20: mol_type = other RNA
tctctgcagatctaaccatt

SEQ ID NO: 18582 - RNA, 20 nt, synthetic construct
  source 1..20: mol_type = other RNA
ttctctgcagatctaaccat

SEQ ID NO: 18583 - RNA, 20 nt, synthetic construct
  source 1..20: mol_type = other RNA
ctgcagagaagagaacacaa

SEQ ID NO: 18584 - RNA, 20 nt, synthetic construct
  source 1..20: mol_type = other RNA
ggttagacagagacatcctc

SEQ ID NO: 18585 - RNA, 20 nt, synthetic construct
  source 1..20: mol_type = other RNA
gttagacagagacatcctca

SEQ ID NO: 18586 - RNA, 20 nt, synthetic construct
  source 1..20: mol_type = other RNA
ttagacagagacatcctcag

SEQ ID NO: 18587 - RNA, 20 nt, synthetic construct
  source 1..20: mol_type = other RNA
tcctcaggggacagctctcc

SEQ ID NO: 18588 - RNA, 20 nt, synthetic construct
  source 1..20: mol_type = other RNA
tcctggagagctgtcccctg

SEQ ID NO: 18589 - RNA, 20 nt, synthetic construct
  source 1..20: mol_type = other RNA
gagaactcatcactggctcc

SEQ ID NO: 18590 - RNA, 20 nt, synthetic construct
  source 1..20: mol_type = other RNA
aaaagcagagaactcatcac

SEQ ID NO: 18591 - RNA, 20 nt, synthetic construct
  source 1..20: mol_type = other RNA
ggtagtttatttacagtcag

SEQ ID NO: 18592 - RNA, 20 nt, synthetic construct
  source 1..20: mol_type = other RNA
tttacagtcagaggcagcat

SEQ ID NO: 18593 - RNA, 20 nt, synthetic construct
  source 1..20: mol_type = other RNA
ttacagtcagaggcagcatt

SEQ ID NO: 18594 - RNA, 20 nt, synthetic construct
  source 1..20: mol_type = other RNA
tacagtcagaggcagcattg

SEQ ID NO: 18595 - RNA, 20 nt, synthetic construct
  source 1..20: mol_type = other RNA
agtcagaggcagcattgggg

SEQ ID NO: 18596 - RNA, 20 nt, synthetic construct
  source 1..20: mol_type = other RNA
gtcagaggcagcattggggt

SEQ ID NO: 18597 - RNA, 20 nt, synthetic construct
  source 1..20: mol_type = other RNA
gaggcagcattggggtggga

SEQ ID NO: 18598 - RNA, 20 nt, synthetic construct
  source 1..20: mol_type = other RNA
gggtgggaaggacgctgagt

SEQ ID NO: 18599 - RNA, 20 nt, synthetic construct
  source 1..20: mol_type = other RNA
aaggacgctgagttggaatc

SEQ ID NO: 18600 - RNA, 20 nt, synthetic construct
  source 1..20: mol_type = other RNA
gacgctgagttggaatctgg

SEQ ID NO: 18601 - RNA, 20 nt, synthetic construct
  source 1..20: mol_type = other RNA
gctgagttggaatctggagg

SEQ ID NO: 18602 - RNA, 20 nt, synthetic construct
  source 1..20: mol_type = other RNA
gtatgtgatgtgtgagattc

SEQ ID NO: 18603 - RNA, 20 nt, synthetic construct
  source 1..20: mol_type = other RNA
tatgtgatgtgtgagattca

SEQ ID NO: 18604 - RNA, 20 nt, synthetic construct
  source 1..20: mol_type = other RNA
agattcagggagagtgcgag

SEQ ID NO: 18605 - RNA, 20 nt, synthetic construct
  source 1..20: mol_type = other RNA
tgtctcaccgttgttgtcgc

SEQ ID NO: 18606 - RNA, 20 nt, synthetic construct
  source 1..20: mol_type = other RNA
tgttgtcgctggacatgagc

SEQ ID NO: 18607 - RNA, 20 nt, synthetic construct
  source 1..20: mol_type = other RNA
ctcatgtccagcgacaacaa

SEQ ID NO: 18608 - RNA, 20 nt, synthetic construct
  source 1..20: mol_type = other RNA
tggacatgagctggtaagtc

SEQ ID NO: 18609 - RNA, 20 nt, synthetic construct
  source 1..20: mol_type = other RNA
gctggtaagtcaggagcttc

SEQ ID NO: 18610 - RNA, 20 nt, synthetic construct
  source 1..20: mol_type = other RNA
ctggtaagtcaggagcttct

SEQ ID NO: 18611 - RNA, 20 nt, synthetic construct
  source 1..20: mol_type = other RNA
cttctgggccttcaagttgt

SEQ ID NO: 18612 - RNA, 20 nt, synthetic construct
  source 1..20: mol_type = other RNA
ggccttcaagttgtaggctc

SEQ ID NO: 18613 - RNA, 20 nt, synthetic construct
  source 1..20: mol_type = other RNA
ggccggagcctacaacttga

SEQ ID NO: 18614 - RNA, 20 nt, synthetic construct
  source 1..20: mol_type = other RNA
gtaggctccggccagattca

SEQ ID NO: 18615 - RNA, 20 nt, synthetic construct
  source 1..20: mol_type = other RNA
cggccagattcatggcaatc

SEQ ID NO: 18616 - RNA, 20 nt, synthetic construct
  source 1..20: mol_type = other RNA
ctgattgccatgaatctggc

SEQ ID NO: 18617 - RNA, 20 nt, synthetic construct
  source 1..20: mol_type = other RNA
attcatggcaatcaggatgc

SEQ ID NO: 18618 - RNA, 20 nt, synthetic construct
  source 1..20: mol_type = other RNA
ttcatggcaatcaggatgct

SEQ ID NO: 18619 - RNA, 20 nt, synthetic construct
  source 1..20: mol_type = other RNA
tcatggcaatcaggatgctg

SEQ ID NO: 18620 - RNA, 20 nt, synthetic construct
  source 1..20: mol_type = other RNA
gcaatcaggatgctggggtt

SEQ ID NO: 18621 - RNA, 20 nt, synthetic construct
  source 1..20: mol_type = other RNA
caatcaggatgctggggttt

SEQ ID NO: 18622 - RNA, 20 nt, synthetic construct
  source 1..20: mol_type = other RNA
caggatgctggggtttgggt

SEQ ID NO: 18623 - RNA, 20 nt, synthetic construct
  source 1..20: mol_type = other RNA
acaagtactcatggagaact

SEQ ID NO: 18624 - RNA, 20 nt, synthetic construct
  source 1..20: mol_type = other RNA
caatggaatacaagtactca

SEQ ID NO: 18625 - RNA, 20 nt, synthetic construct
  source 1..20: mol_type = other RNA
tacttgtattccattgacca

SEQ ID NO: 18626 - RNA, 20 nt, synthetic construct
  source 1..20: mol_type = other RNA
acttgtattccattgaccaa

SEQ ID NO: 18627 - RNA, 20 nt, synthetic construct
  source 1..20: mol_type = other RNA
gaccaagggctcctgtgctg

SEQ ID NO: 18628 - RNA, 20 nt, synthetic construct
  source 1..20: mol_type = other RNA
accaagggctcctgtgctga

SEQ ID NO: 18629 - RNA, 20 nt, synthetic construct
  source 1..20: mol_type = other RNA
gggctcctgtgctgagggaa

SEQ ID NO: 18630 - RNA, 20 nt, synthetic construct
  source 1..20: mol_type = other RNA
tccctcagcacaggagccct

SEQ ID NO: 18631 - RNA, 20 nt, synthetic construct
  source 1..20: mol_type = other RNA
ctcagccgttccctcagcac

SEQ ID NO: 18632 - RNA, 20 nt, synthetic construct
  source 1..20: mol_type = other RNA
ctgagggaacggctgagaag

SEQ ID NO: 18633 - RNA, 20 nt, synthetic construct
  source 1..20: mol_type = other RNA
agggttagaaggtgagtaaa

SEQ ID NO: 18634 - RNA, 20 nt, synthetic construct
  source 1..20: mol_type = other RNA
gagaaggaatgagggttaga

SEQ ID NO: 18635 - RNA, 20 nt, synthetic construct
  source 1..20: mol_type = other RNA
atgtttttgagaaggaatga

SEQ ID NO: 18636 - RNA, 20 nt, synthetic construct
  source 1..20: mol_type = other RNA
aatgtttttgagaaggaatg

SEQ ID NO: 18637 - RNA, 20 nt, synthetic construct
  source 1..20: mol_type = other RNA
cggggataatgtttttgaga

SEQ ID NO: 18638 - RNA, 20 nt, synthetic construct
  source 1..20: mol_type = other RNA
gaaaaagcatcaaagacacg

SEQ ID NO: 18639 - RNA, 20 nt, synthetic construct
  source 1..20: mol_type = other RNA
agaaaaagcatcaaagacac

SEQ ID NO: 18640 - RNA, 20 nt, synthetic construct
  source 1..20: mol_type = other RNA
aagaaaaagcatcaaagaca

SEQ ID NO: 18641 - RNA, 20 nt, synthetic construct
  source 1..20: mol_type = other RNA
cactataggaattccaaaat

SEQ ID NO: 18642 - RNA, 20 nt, synthetic construct
  source 1..20: mol_type = other RNA
tcactataggaattccaaaa

SEQ ID NO: 18643 - RNA, 20 nt, synthetic construct
  source 1..20: mol_type = other RNA
ttgaaaatagcaatcactat

SEQ ID NO: 18644 - RNA, 20 nt, synthetic construct
  source 1..20: mol_type = other RNA
tttcaaccactcagtgtcag

SEQ ID NO: 18645 - RNA, 20 nt, synthetic construct
  source 1..20: mol_type = other RNA
ctgtgacctctgacactgag

SEQ ID NO: 18646 - RNA, 20 nt, synthetic construct
  source 1..20: mol_type = other RNA
gaggtcacagccccttcccc

SEQ ID NO: 18647 - RNA, 20 nt, synthetic construct
  source 1..20: mol_type = other RNA
aggtcacagccccttcccca

SEQ ID NO: 18648 - RNA, 20 nt, synthetic construct
  source 1..20: mol_type = other RNA
aagcagttgccctggggaag

SEQ ID NO: 18649 - RNA, 20 nt, synthetic construct
  source 1..20: mol_type = other RNA
gaagcagttgccctggggaa

SEQ ID NO: 18650 - RNA, 20 nt, synthetic construct
  source 1..20: mol_type = other RNA
ggaagcagttgccctgggga

SEQ ID NO: 18651 - RNA, 20 nt, synthetic construct
  source 1..20: mol_type = other RNA
tcagggaagcagttgccctg

SEQ ID NO: 18652 - RNA, 20 nt, synthetic construct
  source 1..20: mol_type = other RNA
gtcagggaagcagttgccct

SEQ ID NO: 18653 - RNA, 20 nt, synthetic construct
  source 1..20: mol_type = other RNA
ggtcagggaagcagttgccc

SEQ ID NO: 18654 - RNA, 20 nt, synthetic construct
  source 1..20: mol_type = other RNA
aactgcttccctgacctcct

SEQ ID NO: 18655 - RNA, 20 nt, synthetic construct
  source 1..20: mol_type = other RNA
atgtttttccaaggaggtca

SEQ ID NO: 18656 - RNA, 20 nt, synthetic construct
  source 1..20: mol_type = other RNA
gatgtttttccaaggaggtc

SEQ ID NO: 18657 - RNA, 20 nt, synthetic construct
  source 1..20: mol_type = other RNA
agtatgatgtttttccaagg

SEQ ID NO: 18658 - RNA, 20 nt, synthetic construct
  source 1..20: mol_type = other RNA
gtgagtatgatgtttttcca

SEQ ID NO: 18659 - RNA, 20 nt, synthetic construct
  source 1..20: mol_type = other RNA
catactcacagcatgaactc

SEQ ID NO: 18660 - RNA, 20 nt, synthetic construct
  source 1..20: mol_type = other RNA
atactcacagcatgaactct

SEQ ID NO: 18661 - RNA, 20 nt, synthetic construct
  source 1..20: mol_type = other RNA
cacagcatgaactctgggtc

SEQ ID NO: 18662 - RNA, 20 nt, synthetic construct
  source 1..20: mol_type = other RNA
acagcatgaactctgggtct

SEQ ID NO: 18663 - RNA, 20 nt, synthetic construct
  source 1..20: mol_type = other RNA
tcccagctgtagcccagaga

SEQ ID NO: 18664 - RNA, 20 nt, synthetic construct
  source 1..20: mol_type = other RNA
ctgtagcccagagaaggctc

SEQ ID NO: 18665 - RNA, 20 nt, synthetic construct
  source 1..20: mol_type = other RNA
agccttctctgggctacagc

SEQ ID NO: 18666 - RNA, 20 nt, synthetic construct
  source 1..20: mol_type = other RNA
tagcccagagaaggctcagg

SEQ ID NO: 18667 - RNA, 20 nt, synthetic construct
  source 1..20: mol_type = other RNA
agagaaggctcaggaggtag

SEQ ID NO: 18668 - RNA, 20 nt, synthetic construct
  source 1..20: mol_type = other RNA
gagaaggctcaggaggtaga

SEQ ID NO: 18669 - RNA, 20 nt, synthetic construct
  source 1..20: mol_type = other RNA
ctacctcctgagccttctct

SEQ ID NO: 18670 - RNA, 20 nt, synthetic construct
  source 1..20: mol_type = other RNA
tctacctcctgagccttctc

SEQ ID NO: 18671 - RNA, 20 nt, synthetic construct
  source 1..20: mol_type = other RNA
caggaggtagagggcaaacc

SEQ ID NO: 18672 - RNA, 20 nt, synthetic construct
  source 1..20: mol_type = other RNA
gacgagagagtgagatggcc

SEQ ID NO: 18673 - RNA, 20 nt, synthetic construct
  source 1..20: mol_type = other RNA
acatagacgagagagtgaga

SEQ ID NO: 18674 - RNA, 20 nt, synthetic construct
  source 1..20: mol_type = other RNA
cgtctatgtctctcatccac

SEQ ID NO: 18675 - RNA, 20 nt, synthetic construct
  source 1..20: mol_type = other RNA
caggtaccgcgatttgcaag

SEQ ID NO: 18676 - RNA, 20 nt, synthetic construct
  source 1..20: mol_type = other RNA
cttgcaaatcgcggtacctg

SEQ ID NO: 18677 - RNA, 20 nt, synthetic construct
  source 1..20: mol_type = other RNA
aatattccacttgcaaatcg

SEQ ID NO: 18678 - RNA, 20 nt, synthetic construct
  source 1..20: mol_type = other RNA
agggaagcacatataagaga

SEQ ID NO: 18679 - RNA, 20 nt, synthetic construct
  source 1..20: mol_type = other RNA
gggacagattatttaacaaa

SEQ ID NO: 18680 - RNA, 20 nt, synthetic construct
  source 1..20: mol_type = other RNA
ggggacagattatttaacaa

SEQ ID NO: 18681 - RNA, 20 nt, synthetic construct
  source 1..20: mol_type = other RNA
agttaggagaggctgggttg

SEQ ID NO: 18682 - RNA, 20 nt, synthetic construct
  source 1..20: mol_type = other RNA
cagttaggagaggctgggtt

SEQ ID NO: 18683 - RNA, 20 nt, synthetic construct
  source 1..20: mol_type = other RNA
gcagttaggagaggctgggt

SEQ ID NO: 18684 - RNA, 20 nt, synthetic construct
  source 1..20: mol_type = other RNA
aggggcagttaggagaggct

SEQ ID NO: 18685 - RNA, 20 nt, synthetic construct
  source 1..20: mol_type = other RNA
caggggcagttaggagaggc

SEQ ID NO: 18686 - RNA, 20 nt, synthetic construct
  source 1..20: mol_type = other RNA
agcacaggggcagttaggag

SEQ ID NO: 18687 - RNA, 20 nt, synthetic construct
  source 1..20: mol_type = other RNA
aggtcagcacaggggcagtt

SEQ ID NO: 18688 - RNA, 20 nt, synthetic construct
  source 1..20: mol_type = other RNA
gaaaggagaggtcagcacag

SEQ ID NO: 18689 - RNA, 20 nt, synthetic construct
  source 1..20: mol_type = other RNA
ggaaaggagaggtcagcaca

SEQ ID NO: 18690 - RNA, 20 nt, synthetic construct
  source 1..20: mol_type = other RNA
aggaaaggagaggtcagcac

SEQ ID NO: 18691 - RNA, 20 nt, synthetic construct
  source 1..20: mol_type = other RNA
tacttgtatcaggaaaggag

SEQ ID NO: 18692 - RNA, 20 nt, synthetic construct
  source 1..20: mol_type = other RNA
ttacttacttgtatcaggaa

SEQ ID NO: 18693 - RNA, 20 nt, synthetic construct
  source 1..20: mol_type = other RNA
aaaatttacttacttgtatc

SEQ ID NO: 18694 - RNA, 20 nt, synthetic construct
  source 1..20: mol_type = other RNA
taccgactatagaccctcca

SEQ ID NO: 18695 - RNA, 20 nt, synthetic construct
  source 1..20: mol_type = other RNA
caccttggagggtctatagt

SEQ ID NO: 18696 - RNA, 20 nt, synthetic construct
  source 1..20: mol_type = other RNA
agaccctccaaggtgtctga

SEQ ID NO: 18697 - RNA, 20 nt, synthetic construct
  source 1..20: mol_type = other RNA
tcaccttcagacaccttgga

SEQ ID NO: 18698 - RNA, 20 nt, synthetic construct
  source 1..20: mol_type = other RNA
gtcaccttcagacaccttgg

SEQ ID NO: 18699 - RNA, 20 nt, synthetic construct
  source 1..20: mol_type = other RNA
ggtgtctgaaggtgacttct

SEQ ID NO: 18700 - RNA, 20 nt, synthetic construct
  source 1..20: mol_type = other RNA
gaagtcaccttcagacacct

SEQ ID NO: 18701 - RNA, 20 nt, synthetic construct
  source 1..20: mol_type = other RNA
gcacagtcatatgagaaacc

SEQ ID NO: 18702 - RNA, 20 nt, synthetic construct
  source 1..20: mol_type = other RNA
cacagtcatatgagaaacct

SEQ ID NO: 18703 - RNA, 20 nt, synthetic construct
  source 1..20: mol_type = other RNA
acagtcatatgagaaacctg

SEQ ID NO: 18704 - RNA, 20 nt, synthetic construct
  source 1..20: mol_type = other RNA
tcatatgagaaacctggggc

SEQ ID NO: 18705 - RNA, 20 nt, synthetic construct
  source 1..20: mol_type = other RNA
catatgagaaacctggggct

SEQ ID NO: 18706 - RNA, 20 nt, synthetic construct
  source 1..20: mol_type = other RNA
tggggctgggtatgcagtga

SEQ ID NO: 18707 - RNA, 20 nt, synthetic construct
  source 1..20: mol_type = other RNA
ttcactgcatacccagcccc

SEQ ID NO: 18708 - RNA, 20 nt, synthetic construct
  source 1..20: mol_type = other RNA
gagaaaatgtcctttaccaa

SEQ ID NO: 18709 - RNA, 20 nt, synthetic construct
  source 1..20: mol_type = other RNA
aatgtcctttaccaaaggcc

SEQ ID NO: 18710 - RNA, 20 nt, synthetic construct
  source 1..20: mol_type = other RNA
atgtcctttaccaaaggcct

SEQ ID NO: 18711 - RNA, 20 nt, synthetic construct
  source 1..20: mol_type = other RNA
ctgacccaggcctttggtaa

SEQ ID NO: 18712 - RNA, 20 nt, synthetic construct
  source 1..20: mol_type = other RNA
aaaggcctgggtcagacatc

SEQ ID NO: 18713 - RNA, 20 nt, synthetic construct
  source 1..20: mol_type = other RNA
tgatgtctgacccaggcctt

SEQ ID NO: 18714 - RNA, 20 nt, synthetic construct
  source 1..20: mol_type = other RNA
gggtcagacatcaggaagtt

SEQ ID NO: 18715 - RNA, 20 nt, synthetic construct
  source 1..20: mol_type = other RNA
aacttcctgatgtctgaccc

SEQ ID NO: 18716 - RNA, 20 nt, synthetic construct
  source 1..20: mol_type = other RNA
gatacaataagggctagaag

SEQ ID NO: 18717 - RNA, 20 nt, synthetic construct
  source 1..20: mol_type = other RNA
attgtatccaatcagttacc

SEQ ID NO: 18718 - RNA, 20 nt, synthetic construct
  source 1..20: mol_type = other RNA
gtaactgattggatacaata

SEQ ID NO: 18719 - RNA, 20 nt, synthetic construct
  source 1..20: mol_type = other RNA
aaagcagcctggtaactgat

SEQ ID NO: 18720 - RNA, 20 nt, synthetic construct
  source 1..20: mol_type = other RNA
gtagttactaaaaagcagcc

SEQ ID NO: 18721 - RNA, 20 nt, synthetic construct
  source 1..20: mol_type = other RNA
ctttttagtaactacttcac

SEQ ID NO: 18722 - RNA, 20 nt, synthetic construct
  source 1..20: mol_type = other RNA
tttttagtaactacttcact

SEQ ID NO: 18723 - RNA, 20 nt, synthetic construct
  source 1..20: mol_type = other RNA
taactacttcactgggattt

SEQ ID NO: 18724 - RNA, 20 nt, synthetic construct
  source 1..20: mol_type = other RNA
ctgggatttaggccattcat

SEQ ID NO: 18725 - RNA, 20 nt, synthetic construct
  source 1..20: mol_type = other RNA
aatgagctgatgcctatgaa

SEQ ID NO: 18726 - RNA, 20 nt, synthetic construct
  source 1..20: mol_type = other RNA
atgttgtaaagcaggtgtct

SEQ ID NO: 18727 - RNA, 20 nt, synthetic construct
  source 1..20: mol_type = other RNA
gctttacaacatgtcctttt

SEQ ID NO: 18728 - RNA, 20 nt, synthetic construct
  source 1..20: mol_type = other RNA
aaaaggacatgttgtaaagc

SEQ ID NO: 18729 - RNA, 20 nt, synthetic construct
  source 1..20: mol_type = other RNA
acatgtccttttaggctctc

SEQ ID NO: 18730 - RNA, 20 nt, synthetic construct
  source 1..20: mol_type = other RNA
gtccttttaggctctcaggc

SEQ ID NO: 18731 - RNA, 20 nt, synthetic construct
  source 1..20: mol_type = other RNA
tccttttaggctctcaggca

SEQ ID NO: 18732 - RNA, 20 nt, synthetic construct
  source 1..20: mol_type = other RNA
tccctgcctgagagcctaaa

SEQ ID NO: 18733 - RNA, 20 nt, synthetic construct
  source 1..20: mol_type = other RNA
ctctcaggcagggatctgcc

SEQ ID NO: 18734 - RNA, 20 nt, synthetic construct
  source 1..20: mol_type = other RNA
gggatctgccaggtgacatc

SEQ ID NO: 18735 - RNA, 20 nt, synthetic construct
  source 1..20: mol_type = other RNA
tcacaaagccagatgtcacc

SEQ ID NO: 18736 - RNA, 20 nt, synthetic construct
  source 1..20: mol_type = other RNA
tgaaattaatgatgtctacc

SEQ ID NO: 18737 - RNA, 20 nt, synthetic construct
  source 1..20: mol_type = other RNA
taatgatgtctacctggacc

SEQ ID NO: 18738 - RNA, 20 nt, synthetic construct
  source 1..20: mol_type = other RNA
ctaggctagaatccaggtcc

SEQ ID NO: 18739 - RNA, 20 nt, synthetic construct
  source 1..20: mol_type = other RNA
aagagtctaggctagaatcc

SEQ ID NO: 18740 - RNA, 20 nt, synthetic construct
  source 1..20: mol_type = other RNA
caaacaacttcaaagagtct

SEQ ID NO: 18741 - RNA, 20 nt, synthetic construct
  source 1..20: mol_type = other RNA
ctttgaagttgtttgacttt

SEQ ID NO: 18742 - RNA, 20 nt, synthetic construct
  source 1..20: mol_type = other RNA
gtttgactttaggcaagaaa

SEQ ID NO: 18743 - RNA, 20 nt, synthetic construct
  source 1..20: mol_type = other RNA
tttaggcaagaaatggacct

SEQ ID NO: 18744 - RNA, 20 nt, synthetic construct
  source 1..20: mol_type = other RNA
ggacctcggtttcccagaaa

SEQ ID NO: 18745 - RNA, 20 nt, synthetic construct
  source 1..20: mol_type = other RNA
aaaccatttctgggaaaccg

SEQ ID NO: 18746 - RNA, 20 nt, synthetic construct
  source 1..20: mol_type = other RNA
aatcaaacaaaaccatttct

SEQ ID NO: 18747 - RNA, 20 nt, synthetic construct
  source 1..20: mol_type = other RNA
aaatcaaacaaaaccatttc

SEQ ID NO: 18748 - RNA, 20 nt, synthetic construct
  source 1..20: mol_type = other RNA
ttgatttctctttccttatc

SEQ ID NO: 18749 - RNA, 20 nt, synthetic construct
  source 1..20: mol_type = other RNA
atggcttttatctccagata

SEQ ID NO: 18750 - RNA, 20 nt, synthetic construct
  source 1..20: mol_type = other RNA
aaagctttgggtgtttgaga

SEQ ID NO: 18751 - RNA, 20 nt, synthetic construct
  source 1..20: mol_type = other RNA
agataatatctgaaagcttt

SEQ ID NO: 18752 - RNA, 20 nt, synthetic construct
  source 1..20: mol_type = other RNA
aagataatatctgaaagctt

SEQ ID NO: 18753 - RNA, 20 nt, synthetic construct
  source 1..20: mol_type = other RNA
tctgaaatatgtattcttaa

SEQ ID NO: 18754 - RNA, 20 nt, synthetic construct
  source 1..20: mol_type = other RNA
gcaaattatacttctttata

SEQ ID NO: 18755 - RNA, 20 nt, synthetic construct
  source 1..20: mol_type = other RNA
caaattatacttctttataa

SEQ ID NO: 18756 - RNA, 20 nt, synthetic construct
  source 1..20: mol_type = other RNA
ttataagggagaactgaaaa

SEQ ID NO: 18757 - RNA, 20 nt, synthetic construct
  source 1..20: mol_type = other RNA
tatgttgaaattataaagaa

SEQ ID NO: 18758 - RNA, 20 nt, synthetic construct
  source 1..20: mol_type = other RNA
aaatgagctactttacatgc

SEQ ID NO: 18759 - RNA, 20 nt, synthetic construct
  source 1..20: mol_type = other RNA
tgtaaagtagctcattttaa

SEQ ID NO: 18760 - RNA, 20 nt, synthetic construct
  source 1..20: mol_type = other RNA
gtaaagtagctcattttaag

SEQ ID NO: 18761 - RNA, 20 nt, synthetic construct
  source 1..20: mol_type = other RNA
tttaaggggatattctccag

SEQ ID NO: 18762 - RNA, 20 nt, synthetic construct
  source 1..20: mol_type = other RNA
tatgctaagatgggcgccac

SEQ ID NO: 18763 - RNA, 20 nt, synthetic construct
  source 1..20: mol_type = other RNA
tttgacttttatgctaagat

SEQ ID NO: 18764 - RNA, 20 nt, synthetic construct
  source 1..20: mol_type = other RNA
ctttgacttttatgctaaga

SEQ ID NO: 18765 - RNA, 20 nt, synthetic construct
  source 1..20: mol_type = other RNA
ggtcttataggtcatgaaaa

SEQ ID NO: 18766 - RNA, 20 nt, synthetic construct
  source 1..20: mol_type = other RNA
aggtcttataggtcatgaaa

SEQ ID NO: 18767 - RNA, 20 nt, synthetic construct
  source 1..20: mol_type = other RNA
ctataagaccttagaagatc

SEQ ID NO: 18768 - RNA, 20 nt, synthetic construct
  source 1..20: mol_type = other RNA
cagatcttctaaggtcttat

SEQ ID NO: 18769 - RNA, 20 nt, synthetic construct
  source 1..20: mol_type = other RNA
accttagaagatctggctcc

SEQ ID NO: 18770 - RNA, 20 nt, synthetic construct
  source 1..20: mol_type = other RNA
accaggagccagatcttcta

SEQ ID NO: 18771 - RNA, 20 nt, synthetic construct
  source 1..20: mol_type = other RNA
ctgaggtcagaaaggaaacc

SEQ ID NO: 18772 - RNA, 20 nt, synthetic construct
  source 1..20: mol_type = other RNA
tcctttctgacctcagctcc

SEQ ID NO: 18773 - RNA, 20 nt, synthetic construct
  source 1..20: mol_type = other RNA
gcctggagctgaggtcagaa

SEQ ID NO: 18774 - RNA, 20 nt, synthetic construct
  source 1..20: mol_type = other RNA
ggggaaaacgcctggagctg

SEQ ID NO: 18775 - RNA, 20 nt, synthetic construct
  source 1..20: mol_type = other RNA
tgagcaaaggggaaaacgcc

SEQ ID NO: 18776 - RNA, 20 nt, synthetic construct
  source 1..20: mol_type = other RNA
tgggagcggtgtgagcaaag

SEQ ID NO: 18777 - RNA, 20 nt, synthetic construct
  source 1..20: mol_type = other RNA
atgggagcggtgtgagcaaa

SEQ ID NO: 18778 - RNA, 20 nt, synthetic construct
  source 1..20: mol_type = other RNA
gatgggagcggtgtgagcaa

SEQ ID NO: 18779 - RNA, 20 nt, synthetic construct
  source 1..20: mol_type = other RNA
gaagttctgtgtgatgggag

SEQ ID NO: 18780 - RNA, 20 nt, synthetic construct
  source 1..20: mol_type = other RNA
cacaagaagttctgtgtgat

SEQ ID NO: 18781 - RNA, 20 nt, synthetic construct
  source 1..20: mol_type = other RNA
gcacaagaagttctgtgtga

SEQ ID NO: 18782 - RNA, 20 nt, synthetic construct
  source 1..20: mol_type = other RNA
aggtagctgatgtgttcaag

SEQ ID NO: 18783 - RNA, 20 nt, synthetic construct
  source 1..20: mol_type = other RNA
aaggtagctgatgtgttcaa

SEQ ID NO: 18784 - RNA, 20 nt, synthetic construct
  source 1..20: mol_type = other RNA
aaaggtagctgatgtgttca

SEQ ID NO: 18785 - RNA, 20 nt, synthetic construct
  source 1..20: mol_type = other RNA
gagggggacatcatgtgcaa

SEQ ID NO: 18786 - RNA, 20 nt, synthetic construct
  source 1..20: mol_type = other RNA
catgatgtccccctcagccc

SEQ ID NO: 18787 - RNA, 20 nt, synthetic construct
  source 1..20: mol_type = other RNA
aagagggtcctgggctgagg

SEQ ID NO: 18788 - RNA, 20 nt, synthetic construct
  source 1..20: mol_type = other RNA
gaagagggtcctgggctgag

SEQ ID NO: 18789 - RNA, 20 nt, synthetic construct
  source 1..20: mol_type = other RNA
agaagagggtcctgggctga

SEQ ID NO: 18790 - RNA, 20 nt, synthetic construct
  source 1..20: mol_type = other RNA
aagaagagggtcctgggctg

SEQ ID NO: 18791 - RNA, 20 nt, synthetic construct
  source 1..20: mol_type = other RNA
atttaaaagaagagggtcct

SEQ ID NO: 18792 - RNA, 20 nt, synthetic construct
  source 1..20: mol_type = other RNA
tatttaaaagaagagggtcc

SEQ ID NO: 18793 - RNA, 20 nt, synthetic construct
  source 1..20: mol_type = other RNA
tcttcttttaaatagcctca

SEQ ID NO: 18794 - RNA, 20 nt, synthetic construct
  source 1..20: mol_type = other RNA
tgaggctatttaaaagaaga

SEQ ID NO: 18795 - RNA, 20 nt, synthetic construct
  source 1..20: mol_type = other RNA
atgaggctatttaaaagaag

SEQ ID NO: 18796 - RNA, 20 nt, synthetic construct
  source 1..20: mol_type = other RNA
gatgtgaggaagccaccatg

SEQ ID NO: 18797 - RNA, 20 nt, synthetic construct
  source 1..20: mol_type = other RNA
gcagagacatgaaggatgtg

SEQ ID NO: 18798 - RNA, 20 nt, synthetic construct
  source 1..20: mol_type = other RNA
tccttcatgtctctgctcag

SEQ ID NO: 18799 - RNA, 20 nt, synthetic construct
  source 1..20: mol_type = other RNA
acctctgagcagagacatga

SEQ ID NO: 18800 - RNA, 20 nt, synthetic construct
  source 1..20: mol_type = other RNA
gcttttagagacgccttccc

SEQ ID NO: 18801 - RNA, 20 nt, synthetic construct
  source 1..20: mol_type = other RNA
ttatgtagggtggcctggga

SEQ ID NO: 18802 - RNA, 20 nt, synthetic construct
  source 1..20: mol_type = other RNA
gatcttatgtagggtggcct

SEQ ID NO: 18803 - RNA, 20 nt, synthetic construct
  source 1..20: mol_type = other RNA
ggatcttatgtagggtggcc

SEQ ID NO: 18804 - RNA, 20 nt, synthetic construct
  source 1..20: mol_type = other RNA
atgtaggatcttatgtaggg

SEQ ID NO: 18805 - RNA, 20 nt, synthetic construct
  source 1..20: mol_type = other RNA
aggatgtaggatcttatgta

SEQ ID NO: 18806 - RNA, 20 nt, synthetic construct
  source 1..20: mol_type = other RNA
gaggatgtaggatcttatgt

SEQ ID NO: 18807 - RNA, 20 nt, synthetic construct
  source 1..20: mol_type = other RNA
gtcagtggaggtgaggatgt

SEQ ID NO: 18808 - RNA, 20 nt, synthetic construct
  source 1..20: mol_type = other RNA
gaggggtgtcagtggaggtg

SEQ ID NO: 18809 - RNA, 20 nt, synthetic construct
  source 1..20: mol_type = other RNA
ggcatgaggggtgtcagtgg

SEQ ID NO: 18810 - RNA, 20 nt, synthetic construct
  source 1..20: mol_type = other RNA
aggggcatgaggggtgtcag

SEQ ID NO: 18811 - RNA, 20 nt, synthetic construct
  source 1..20: mol_type = other RNA
tagcaggcgaggggcatgag

SEQ ID NO: 18812 - RNA, 20 nt, synthetic construct
  source 1..20: mol_type = other RNA
atagcaggcgaggggcatga

SEQ ID NO: 18813 - RNA, 20 nt, synthetic construct
  source 1..20: mol_type = other RNA
tatagcaggcgaggggcatg

SEQ ID NO: 18814 - RNA, 20 nt, synthetic construct
  source 1..20: mol_type = other RNA
aatgagttatagcaggcgag

SEQ ID NO: 18815 - RNA, 20 nt, synthetic construct
  source 1..20: mol_type = other RNA
caatgagttatagcaggcga

SEQ ID NO: 18816 - RNA, 20 nt, synthetic construct
  source 1..20: mol_type = other RNA
gcaatgagttatagcaggcg

SEQ ID NO: 18817 - RNA, 20 nt, synthetic construct
  source 1..20: mol_type = other RNA
agagggcaatgagttatagc

SEQ ID NO: 18818 - RNA, 20 nt, synthetic construct
  source 1..20: mol_type = other RNA
cctctgtcgcactaagtgtg

SEQ ID NO: 18819 - RNA, 20 nt, synthetic construct
  source 1..20: mol_type = other RNA
cacacacttagtgcgacaga

SEQ ID NO: 18820 - RNA, 20 nt, synthetic construct
  source 1..20: mol_type = other RNA
ccacacacttagtgcgacag

SEQ ID NO: 18821 - RNA, 20 nt, synthetic construct
  source 1..20: mol_type = other RNA
actagaatgtctgctccacg

SEQ ID NO: 18822 - RNA, 20 nt, synthetic construct
  source 1..20: mol_type = other RNA
gtggagcagacattctagta

SEQ ID NO: 18823 - RNA, 20 nt, synthetic construct
  source 1..20: mol_type = other RNA
cgtggagcagacattctagt

SEQ ID NO: 18824 - RNA, 20 nt, synthetic construct
  source 1..20: mol_type = other RNA
gaatgtctgctccacgaggg

SEQ ID NO: 18825 - RNA, 20 nt, synthetic construct
  source 1..20: mol_type = other RNA
aatgtctgctccacgaggga

SEQ ID NO: 18826 - RNA, 20 nt, synthetic construct
  source 1..20: mol_type = other RNA
atgtctgctccacgagggag

SEQ ID NO: 18827 - RNA, 20 nt, synthetic construct
  source 1..20: mol_type = other RNA
agggaggggctttgtctctt

SEQ ID NO: 18828 - RNA, 20 nt, synthetic construct
  source 1..20: mol_type = other RNA
aggtagtgttgtaagggcta

SEQ ID NO: 18829 - RNA, 20 nt, synthetic construct
  source 1..20: mol_type = other RNA
tgagctaggtagtgttgtaa

SEQ ID NO: 18830 - RNA, 20 nt, synthetic construct
  source 1..20: mol_type = other RNA
gtgagctaggtagtgttgta

SEQ ID NO: 18831 - RNA, 20 nt, synthetic construct
  source 1..20: mol_type = other RNA
ttttatttctactgtgagct

SEQ ID NO: 18832 - RNA, 20 nt, synthetic construct
  source 1..20: mol_type = other RNA
taatgagcaaatgtaagaca

SEQ ID NO: 18833 - RNA, 20 nt, synthetic construct
  source 1..20: mol_type = other RNA
aatgagcaaatgtaagacat

SEQ ID NO: 18834 - RNA, 20 nt, synthetic construct
  source 1..20: mol_type = other RNA
ataaagcattttttccccct

SEQ ID NO: 18835 - RNA, 20 nt, synthetic construct
  source 1..20: mol_type = other RNA
taaagcattttttccccctt

SEQ ID NO: 18836 - RNA, 20 nt, synthetic construct
  source 1..20: mol_type = other RNA
tttttcccccttgggaaaca

SEQ ID NO: 18837 - RNA, 20 nt, synthetic construct
  source 1..20: mol_type = other RNA
ttttcccccttgggaaacat

SEQ ID NO: 18838 - RNA, 20 nt, synthetic construct
  source 1..20: mol_type = other RNA
ctcacccatgtttcccaagg

SEQ ID NO: 18839 - RNA, 20 nt, synthetic construct
  source 1..20: mol_type = other RNA
actcacccatgtttcccaag

SEQ ID NO: 18840 - RNA, 20 nt, synthetic construct
  source 1..20: mol_type = other RNA
aactcacccatgtttcccaa

SEQ ID NO: 18841 - RNA, 20 nt, synthetic construct
  source 1..20: mol_type = other RNA
aaactcacccatgtttccca

SEQ ID NO: 18842 - RNA, 20 nt, synthetic construct
  source 1..20: mol_type = other RNA
gttttgtgagatgagagcac

SEQ ID NO: 18843 - RNA, 20 nt, synthetic construct
  source 1..20: mol_type = other RNA
ttttgtgagatgagagcaca

SEQ ID NO: 18844 - RNA, 20 nt, synthetic construct
  source 1..20: mol_type = other RNA
tgagagcacagggtacatac

SEQ ID NO: 18845 - RNA, 20 nt, synthetic construct
  source 1..20: mol_type = other RNA
gagagcacagggtacatact

SEQ ID NO: 18846 - RNA, 20 nt, synthetic construct
  source 1..20: mol_type = other RNA
agagcacagggtacatactg

SEQ ID NO: 18847 - RNA, 20 nt, synthetic construct
  source 1..20: mol_type = other RNA
gggtacatactggggtgtgc

SEQ ID NO: 18848 - RNA, 20 nt, synthetic construct
  source 1..20: mol_type = other RNA
gtgctggacaacttctaaca

SEQ ID NO: 18849 - RNA, 20 nt, synthetic construct
  source 1..20: mol_type = other RNA
taccgggaggtgaaaacaca

SEQ ID NO: 18850 - RNA, 20 nt, synthetic construct
  source 1..20: mol_type = other RNA
ataccgggaggtgaaaacac

SEQ ID NO: 18851 - RNA, 20 nt, synthetic construct
  source 1..20: mol_type = other RNA
ttattcagataaaatattat

SEQ ID NO: 18852 - RNA, 20 nt, synthetic construct
  source 1..20: mol_type = other RNA
gtttgtattttgcatactca

SEQ ID NO: 18853 - RNA, 20 nt, synthetic construct
  source 1..20: mol_type = other RNA
aaagtaaaatgaacattttg

SEQ ID NO: 18854 - RNA, 20 nt, synthetic construct
  source 1..20: mol_type = other RNA
tttatattacatatttatta

SEQ ID NO: 18855 - RNA, 20 nt, synthetic construct
  source 1..20: mol_type = other RNA
attacatatttattaaggca

SEQ ID NO: 18856 - RNA, 20 nt, synthetic construct
  source 1..20: mol_type = other RNA
aaacacatttgttctgctta

SEQ ID NO: 18857 - RNA, 20 nt, synthetic construct
  source 1..20: mol_type = other RNA
tgttctgcttaaggcatact

SEQ ID NO: 18858 - RNA, 20 nt, synthetic construct
  source 1..20: mol_type = other RNA
gttctgcttaaggcatactt

SEQ ID NO: 18859 - RNA, 20 nt, synthetic construct
  source 1..20: mol_type = other RNA
atgtgcaataatttgtacaa

SEQ ID NO: 18860 - RNA, 20 nt, synthetic construct
  source 1..20: mol_type = other RNA
agacagtctgttatgcactg

SEQ ID NO: 18861 - RNA, 20 nt, synthetic construct
  source 1..20: mol_type = other RNA
aaatgctaaagaagtaaacc

SEQ ID NO: 18862 - RNA, 20 nt, synthetic construct
  source 1..20: mol_type = other RNA
ccaggtatattacctgactt

SEQ ID NO: 18863 - RNA, 20 nt, synthetic construct
  source 1..20: mol_type = other RNA
cctaagtcaggtaatatacc

SEQ ID NO: 18864 - RNA, 20 nt, synthetic construct
  source 1..20: mol_type = other RNA
caacatttatgacctaagtc

SEQ ID NO: 18865 - RNA, 20 nt, synthetic construct
  source 1..20: mol_type = other RNA
aactgctgcatactttgaca

SEQ ID NO: 18866 - RNA, 20 nt, synthetic construct
  source 1..20: mol_type = other RNA
atgcagcagtttgaaaactt

SEQ ID NO: 18867 - RNA, 20 nt, synthetic construct
  source 1..20: mol_type = other RNA
aaaactttggcttccttgtt

SEQ ID NO: 18868 - RNA, 20 nt, synthetic construct
  source 1..20: mol_type = other RNA
ggttctaaaggtaccaaaca

SEQ ID NO: 18869 - RNA, 20 nt, synthetic construct
  source 1..20: mol_type = other RNA
ttggtgagtcttggttctaa

SEQ ID NO: 18870 - RNA, 20 nt, synthetic construct
  source 1..20: mol_type = other RNA
tgatggtgcttggtgagtct

SEQ ID NO: 18871 - RNA, 20 nt, synthetic construct
  source 1..20: mol_type = other RNA
ctcaccaagcaccatcattt

SEQ ID NO: 18872 - RNA, 20 nt, synthetic construct
  source 1..20: mol_type = other RNA
atagcctaaatgatggtgct

SEQ ID NO: 18873 - RNA, 20 nt, synthetic construct
  source 1..20: mol_type = other RNA
tgtttaaatagcctaaatga

SEQ ID NO: 18874 - RNA, 20 nt, synthetic construct
  source 1..20: mol_type = other RNA
agaagaagaggaagaaattc

SEQ ID NO: 18875 - RNA, 20 nt, synthetic construct
  source 1..20: mol_type = other RNA
ttcttctaacatcataataa

SEQ ID NO: 18876 - RNA, 20 nt, synthetic construct
  source 1..20: mol_type = other RNA
tattatgatgttagaagaag

SEQ ID NO: 18877 - RNA, 20 nt, synthetic construct
  source 1..20: mol_type = other RNA
tcataataatggcttttaga

SEQ ID NO: 18878 - RNA, 20 nt, synthetic construct
  source 1..20: mol_type = other RNA
tagaaggtaaagagaataca

SEQ ID NO: 18879 - RNA, 20 nt, synthetic construct
  source 1..20: mol_type = other RNA
ttgcatcaatacacaattca

SEQ ID NO: 18880 - RNA, 20 nt, synthetic construct
  source 1..20: mol_type = other RNA
tgcatcaatacacaattcaa

SEQ ID NO: 18881 - RNA, 20 nt, synthetic construct
  source 1..20: mol_type = other RNA
tacacaattcaagggaattc

SEQ ID NO: 18882 - RNA, 20 nt, synthetic construct
  source 1..20: mol_type = other RNA
gtcttccctcccccaactca

SEQ ID NO: 18883 - RNA, 20 nt, synthetic construct
  source 1..20: mol_type = other RNA
tatatccgtgagttggggga

SEQ ID NO: 18884 - RNA, 20 nt, synthetic construct
  source 1..20: mol_type = other RNA
ttatatccgtgagttggggg

SEQ ID NO: 18885 - RNA, 20 nt, synthetic construct
  source 1..20: mol_type = other RNA
aaattatatccgtgagttgg

SEQ ID NO: 18886 - RNA, 20 nt, synthetic construct
  source 1..20: mol_type = other RNA
taaattatatccgtgagttg

SEQ ID NO: 18887 - RNA, 20 nt, synthetic construct
  source 1..20: mol_type = other RNA
ataaattatatccgtgagtt

SEQ ID NO: 18888 - RNA, 20 nt, synthetic construct
  source 1..20: mol_type = other RNA
tataaattatatccgtgagt

SEQ ID NO: 18889 - RNA, 20 nt, synthetic construct
  source 1..20: mol_type = other RNA
actggaagttgtggatatca

SEQ ID NO: 18890 - RNA, 20 nt, synthetic construct
  source 1..20: mol_type = other RNA
gactggaagttgtggatatc

SEQ ID NO: 18891 - RNA, 20 nt, synthetic construct
  source 1..20: mol_type = other RNA
acaacttccagtcaccccct

SEQ ID NO: 18892 - RNA, 20 nt, synthetic construct
  source 1..20: mol_type = other RNA
aagggggtgactggaagttg

SEQ ID NO: 18893 - RNA, 20 nt, synthetic construct
  source 1..20: mol_type = other RNA
caaaatgccaagggggtgac

SEQ ID NO: 18894 - RNA, 20 nt, synthetic construct
  source 1..20: mol_type = other RNA
ccttggcattttgtaagtcc

SEQ ID NO: 18895 - RNA, 20 nt, synthetic construct
  source 1..20: mol_type = other RNA
ggacttacaaaatgccaagg

SEQ ID NO: 18896 - RNA, 20 nt, synthetic construct
  source 1..20: mol_type = other RNA
tggacttacaaaatgccaag

SEQ ID NO: 18897 - RNA, 20 nt, synthetic construct
  source 1..20: mol_type = other RNA
ctggacttacaaaatgccaa

SEQ ID NO: 18898 - RNA, 20 nt, synthetic construct
  source 1..20: mol_type = other RNA
cctggacttacaaaatgcca

SEQ ID NO: 18899 - RNA, 20 nt, synthetic construct
  source 1..20: mol_type = other RNA
aagtccaggaatattcaagt

SEQ ID NO: 18900 - RNA, 20 nt, synthetic construct
  source 1..20: mol_type = other RNA
aaatccgacttgaatattcc

SEQ ID NO: 18901 - RNA, 20 nt, synthetic construct
  source 1..20: mol_type = other RNA
attcaagtcggatttagaat

SEQ ID NO: 18902 - RNA, 20 nt, synthetic construct
  source 1..20: mol_type = other RNA
gaacagatggggtctgtgac

SEQ ID NO: 18903 - RNA, 20 nt, synthetic construct
  source 1..20: mol_type = other RNA
caaaaatcaaagaacagatg

SEQ ID NO: 18904 - RNA, 20 nt, synthetic construct
  source 1..20: mol_type = other RNA
acaaaaatcaaagaacagat

SEQ ID NO: 18905 - RNA, 20 nt, synthetic construct
  source 1..20: mol_type = other RNA
gacaaaaatcaaagaacaga

SEQ ID NO: 18906 - RNA, 20 nt, synthetic construct
  source 1..20: mol_type = other RNA
gttctttgatttttgtcttt

SEQ ID NO: 18907 - RNA, 20 nt, synthetic construct
  source 1..20: mol_type = other RNA
gtggataatcaggaaaaatg

SEQ ID NO: 18908 - RNA, 20 nt, synthetic construct
  source 1..20: mol_type = other RNA
catcttgtgagtggataatc

SEQ ID NO: 18909 - RNA, 20 nt, synthetic construct
  source 1..20: mol_type = other RNA
cactcacaagatgactcagt

SEQ ID NO: 18910 - RNA, 20 nt, synthetic construct
  source 1..20: mol_type = other RNA
actcacaagatgactcagtt

SEQ ID NO: 18911 - RNA, 20 nt, synthetic construct
  source 1..20: mol_type = other RNA
caactgagtcatcttgtgag

SEQ ID NO: 18912 - RNA, 20 nt, synthetic construct
  source 1..20: mol_type = other RNA
accatgattgtagtgctttc

SEQ ID NO: 18913 - RNA, 20 nt, synthetic construct
  source 1..20: mol_type = other RNA
tgattgtagtgctttctggc

SEQ ID NO: 18914 - RNA, 20 nt, synthetic construct
  source 1..20: mol_type = other RNA
gattgtagtgctttctggct

SEQ ID NO: 18915 - RNA, 20 nt, synthetic construct
  source 1..20: mol_type = other RNA
gccagaaagcactacaatca

SEQ ID NO: 18916 - RNA, 20 nt, synthetic construct
  source 1..20: mol_type = other RNA
ggctgggctccttccctcat

SEQ ID NO: 18917 - RNA, 20 nt, synthetic construct
  source 1..20: mol_type = other RNA
gctgggctccttccctcatc

SEQ ID NO: 18918 - RNA, 20 nt, synthetic construct
  source 1..20: mol_type = other RNA
actgtcttcccgatgaggga

SEQ ID NO: 18919 - RNA, 20 nt, synthetic construct
  source 1..20: mol_type = other RNA
tcacactgtcttcccgatga

SEQ ID NO: 18920 - RNA, 20 nt, synthetic construct
  source 1..20: mol_type = other RNA
ttcacactgtcttcccgatg

SEQ ID NO: 18921 - RNA, 20 nt, synthetic construct
  source 1..20: mol_type = other RNA
aaaaatactgaattctcttc

SEQ ID NO: 18922 - RNA, 20 nt, synthetic construct
  source 1..20: mol_type = other RNA
tgaattctcttctggcagtg

SEQ ID NO: 18923 - RNA, 20 nt, synthetic construct
  source 1..20: mol_type = other RNA
gaattctcttctggcagtgt

SEQ ID NO: 18924 - RNA, 20 nt, synthetic construct
  source 1..20: mol_type = other RNA
tgtgggtcatatccactgtc

SEQ ID NO: 18925 - RNA, 20 nt, synthetic construct
  source 1..20: mol_type = other RNA
gtgggtcatatccactgtct

SEQ ID NO: 18926 - RNA, 20 nt, synthetic construct
  source 1..20: mol_type = other RNA
catttttaaatcccagacag

SEQ ID NO: 18927 - RNA, 20 nt, synthetic construct
  source 1..20: mol_type = other RNA
aaaatgcctcttcatgtgta

SEQ ID NO: 18928 - RNA, 20 nt, synthetic construct
  source 1..20: mol_type = other RNA
gcctcttcatgtgtaaggcg

SEQ ID NO: 18929 - RNA, 20 nt, synthetic construct
  source 1..20: mol_type = other RNA
tcttcatgtgtaaggcgagg

SEQ ID NO: 18930 - RNA, 20 nt, synthetic construct
  source 1..20: mol_type = other RNA
acctcgccttacacatgaag

SEQ ID NO: 18931 - RNA, 20 nt, synthetic construct
  source 1..20: mol_type = other RNA
taaggcgaggtggtccgacc

SEQ ID NO: 18932 - RNA, 20 nt, synthetic construct
  source 1..20: mol_type = other RNA
ggtccgacctggaaaatgct

SEQ ID NO: 18933 - RNA, 20 nt, synthetic construct
  source 1..20: mol_type = other RNA
cgaccgagcattttccaggt

SEQ ID NO: 18934 - RNA, 20 nt, synthetic construct
  source 1..20: mol_type = other RNA
aatgcgaccgagcattttcc

SEQ ID NO: 18935 - RNA, 20 nt, synthetic construct
  source 1..20: mol_type = other RNA
ctcggtcgcatttttggcac

SEQ ID NO: 18936 - RNA, 20 nt, synthetic construct
  source 1..20: mol_type = other RNA
tcgcatttttggcactggaa

SEQ ID NO: 18937 - RNA, 20 nt, synthetic construct
  source 1..20: mol_type = other RNA
cgcatttttggcactggaac

SEQ ID NO: 18938 - RNA, 20 nt, synthetic construct
  source 1..20: mol_type = other RNA
atttttggcactggaacggg

SEQ ID NO: 18939 - RNA, 20 nt, synthetic construct
  source 1..20: mol_type = other RNA
ggcggtgccccgtgtgttta

SEQ ID NO: 18940 - RNA, 20 nt, synthetic construct
  source 1..20: mol_type = other RNA
cgtgtgtttacggtagtgcc

SEQ ID NO: 18941 - RNA, 20 nt, synthetic construct
  source 1..20: mol_type = other RNA
ggcactaccgtaaacacacg

SEQ ID NO: 18942 - RNA, 20 nt, synthetic construct
  source 1..20: mol_type = other RNA
aggcactaccgtaaacacac

SEQ ID NO: 18943 - RNA, 20 nt, synthetic construct
  source 1..20: mol_type = other RNA
caggcactaccgtaaacaca

SEQ ID NO: 18944 - RNA, 20 nt, synthetic construct
  source 1..20: mol_type = other RNA
gcctggtcagttcatctgag

SEQ ID NO: 18945 - RNA, 20 nt, synthetic construct
  source 1..20: mol_type = other RNA
cctggtcagttcatctgagc

SEQ ID NO: 18946 - RNA, 20 nt, synthetic construct
  source 1..20: mol_type = other RNA
cccgctcagatgaactgacc

SEQ ID NO: 18947 - RNA, 20 nt, synthetic construct
  source 1..20: mol_type = other RNA
cacagccgtcccagtcacag

SEQ ID NO: 18948 - RNA, 20 nt, synthetic construct
  source 1..20: mol_type = other RNA
cactgtgactgggacggctg

SEQ ID NO: 18949 - RNA, 20 nt, synthetic construct
  source 1..20: mol_type = other RNA
ccgtcccagtcacagtggta

SEQ ID NO: 18950 - RNA, 20 nt, synthetic construct
  source 1..20: mol_type = other RNA
ccttaccactgtgactggga

SEQ ID NO: 18951 - RNA, 20 nt, synthetic construct
  source 1..20: mol_type = other RNA
gaaaccttaccactgtgact

SEQ ID NO: 18952 - RNA, 20 nt, synthetic construct
  source 1..20: mol_type = other RNA
agaaaccttaccactgtgac

SEQ ID NO: 18953 - RNA, 20 nt, synthetic construct
  source 1..20: mol_type = other RNA
gtaaggtttctcacctgtaa

SEQ ID NO: 18954 - RNA, 20 nt, synthetic construct
  source 1..20: mol_type = other RNA
tttttttcttttacctttac

SEQ ID NO: 18955 - RNA, 20 nt, synthetic construct
  source 1..20: mol_type = other RNA
tcgccccttttaaaaactga

SEQ ID NO: 18956 - RNA, 20 nt, synthetic construct
  source 1..20: mol_type = other RNA
tggccttcagtttttaaaag

SEQ ID NO: 18957 - RNA, 20 nt, synthetic construct
  source 1..20: mol_type = other RNA
ctggccttcagtttttaaaa

SEQ ID NO: 18958 - RNA, 20 nt, synthetic construct
  source 1..20: mol_type = other RNA
tctggccttcagtttttaaa

SEQ ID NO: 18959 - RNA, 20 nt, synthetic construct
  source 1..20: mol_type = other RNA
gtcagagttggtttactatc

SEQ ID NO: 18960 - RNA, 20 nt, synthetic construct
  source 1..20: mol_type = other RNA
ctttaggatagggtcagagt

SEQ ID NO: 18961 - RNA, 20 nt, synthetic construct
  source 1..20: mol_type = other RNA
accctatcctaaagaaatcc

SEQ ID NO: 18962 - RNA, 20 nt, synthetic construct
  source 1..20: mol_type = other RNA
tcctggatttctttaggata

SEQ ID NO: 18963 - RNA, 20 nt, synthetic construct
  source 1..20: mol_type = other RNA
ttcctggatttctttaggat

SEQ ID NO: 18964 - RNA, 20 nt, synthetic construct
  source 1..20: mol_type = other RNA
ccactggtagcctatggggc

SEQ ID NO: 18965 - RNA, 20 nt, synthetic construct
  source 1..20: mol_type = other RNA
ccagccccataggctaccag

SEQ ID NO: 18966 - RNA, 20 nt, synthetic construct
  source 1..20: mol_type = other RNA
tatggggctggaagctaacc

SEQ ID NO: 18967 - RNA, 20 nt, synthetic construct
  source 1..20: mol_type = other RNA
atggggctggaagctaacct

SEQ ID NO: 18968 - RNA, 20 nt, synthetic construct
  source 1..20: mol_type = other RNA
aggttagcttccagccccat

SEQ ID NO: 18969 - RNA, 20 nt, synthetic construct
  source 1..20: mol_type = other RNA
gaagctaacctgggaagtca

SEQ ID NO: 18970 - RNA, 20 nt, synthetic construct
  source 1..20: mol_type = other RNA
gctaacctgggaagtcaagg

SEQ ID NO: 18971 - RNA, 20 nt, synthetic construct
  source 1..20: mol_type = other RNA
gggaagtcaaggaggcactg

SEQ ID NO: 18972 - RNA, 20 nt, synthetic construct
  source 1..20: mol_type = other RNA
cagtgcctccttgacttccc

SEQ ID NO: 18973 - RNA, 20 nt, synthetic construct
  source 1..20: mol_type = other RNA
aggcactgaggagtgtccac

SEQ ID NO: 18974 - RNA, 20 nt, synthetic construct
  source 1..20: mol_type = other RNA
gagtgtccactggtagccta

SEQ ID NO: 18975 - RNA, 20 nt, synthetic construct
  source 1..20: mol_type = other RNA
agtgtccactggtagcctat

SEQ ID NO: 18976 - RNA, 20 nt, synthetic construct
  source 1..20: mol_type = other RNA
gtgtccactggtagcctatg

SEQ ID NO: 18977 - RNA, 20 nt, synthetic construct
  source 1..20: mol_type = other RNA
ccactggtagcctatggggc

SEQ ID NO: 18978 - RNA, 20 nt, synthetic construct
  source 1..20: mol_type = other RNA
ccagccccataggctaccag

SEQ ID NO: 18979 - RNA, 20 nt, synthetic construct
  source 1..20: mol_type = other RNA
gggttagcttccagccccat

SEQ ID NO: 18980 - RNA, 20 nt, synthetic construct
  source 1..20: mol_type = other RNA
acaaactgcagaagggaggg

SEQ ID NO: 18981 - RNA, 20 nt, synthetic construct
  source 1..20: mol_type = other RNA
gacaaactgcagaagggagg

SEQ ID NO: 18982 - RNA, 20 nt, synthetic construct
  source 1..20: mol_type = other RNA
ggacaaactgcagaagggag

SEQ ID NO: 18983 - RNA, 20 nt, synthetic construct
  source 1..20: mol_type = other RNA
gggacaaactgcagaaggga

SEQ ID NO: 18984 - RNA, 20 nt, synthetic construct
  source 1..20: mol_type = other RNA
ggggacaaactgcagaaggg

SEQ ID NO: 18985 - RNA, 20 nt, synthetic construct
  source 1..20: mol_type = other RNA
tagggggacaaactgcagaa

SEQ ID NO: 18986 - RNA, 20 nt, synthetic construct
  source 1..20: mol_type = other RNA
gtagggggacaaactgcaga

SEQ ID NO: 18987 - RNA, 20 nt, synthetic construct
  source 1..20: mol_type = other RNA
agtttgtccccctacctgtg

SEQ ID NO: 18988 - RNA, 20 nt, synthetic construct
  source 1..20: mol_type = other RNA
gtttgtccccctacctgtgt

SEQ ID NO: 18989 - RNA, 20 nt, synthetic construct
  source 1..20: mol_type = other RNA
ccctacctgtgtgggttcgc

SEQ ID NO: 18990 - RNA, 20 nt, synthetic construct
  source 1..20: mol_type = other RNA
tgcgaacccacacaggtagg

SEQ ID NO: 18991 - RNA, 20 nt, synthetic construct
  source 1..20: mol_type = other RNA
ctgcgaacccacacaggtag

SEQ ID NO: 18992 - RNA, 20 nt, synthetic construct
  source 1..20: mol_type = other RNA
cctgcgaacccacacaggta

SEQ ID NO: 18993 - RNA, 20 nt, synthetic construct
  source 1..20: mol_type = other RNA
acctgcgaacccacacaggt

SEQ ID NO: 18994 - RNA, 20 nt, synthetic construct
  source 1..20: mol_type = other RNA
gcacacctgcgaacccacac

SEQ ID NO: 18995 - RNA, 20 nt, synthetic construct
  source 1..20: mol_type = other RNA
ttcgcaggtgtgccttgaga

SEQ ID NO: 18996 - RNA, 20 nt, synthetic construct
  source 1..20: mol_type = other RNA
tcgcaggtgtgccttgagat

SEQ ID NO: 18997 - RNA, 20 nt, synthetic construct
  source 1..20: mol_type = other RNA
gagatgggaactctttgtgt

SEQ ID NO: 18998 - RNA, 20 nt, synthetic construct
  source 1..20: mol_type = other RNA
cacaaagagttcccatctca

SEQ ID NO: 18999 - RNA, 20 nt, synthetic construct
  source 1..20: mol_type = other RNA
agcccgcgtaatcacaagtg

SEQ ID NO: 19000 - RNA, 20 nt, synthetic construct
  source 1..20: mol_type = other RNA
gcccgcgtaatcacaagtgt

SEQ ID NO: 19001 - RNA, 20 nt, synthetic construct
  source 1..20: mol_type = other RNA
cgcgtaatcacaagtgtggg

SEQ ID NO: 19002 - RNA, 20 nt, synthetic construct
  source 1..20: mol_type = other RNA
gtaatcacaagtgtgggtgg

SEQ ID NO: 19003 - RNA, 20 nt, synthetic construct
  source 1..20: mol_type = other RNA
cacccacacttgtgattacg

SEQ ID NO: 19004 - RNA, 20 nt, synthetic construct
  source 1..20: mol_type = other RNA
tgtgggtggcggtccttttc

SEQ ID NO: 19005 - RNA, 20 nt, synthetic construct
  source 1..20: mol_type = other RNA
gtgggtggcggtccttttcc

SEQ ID NO: 19006 - RNA, 20 nt, synthetic construct
  source 1..20: mol_type = other RNA
tgggtggcggtccttttccg

SEQ ID NO: 19007 - RNA, 20 nt, synthetic construct
  source 1..20: mol_type = other RNA
gacgatcgtggccccggaaa

SEQ ID NO: 19008 - RNA, 20 nt, synthetic construct
  source 1..20: mol_type = other RNA
ggggaagacgatcgtggccc

SEQ ID NO: 19009 - RNA, 20 nt, synthetic construct
  source 1..20: mol_type = other RNA
cacgatcgtcttcccctctt

SEQ ID NO: 19010 - RNA, 20 nt, synthetic construct
  source 1..20: mol_type = other RNA
caaagaggggaagacgatcg

SEQ ID NO: 19011 - RNA, 20 nt, synthetic construct
  source 1..20: mol_type = other RNA
tcgtcttcccctctttggct

SEQ ID NO: 19012 - RNA, 20 nt, synthetic construct
  source 1..20: mol_type = other RNA
cgtcttcccctctttggctt

SEQ ID NO: 19013 - RNA, 20 nt, synthetic construct
  source 1..20: mol_type = other RNA
ctctttggcttgggctcctc

SEQ ID NO: 19014 - RNA, 20 nt, synthetic construct
  source 1..20: mol_type = other RNA
gaggagcccaagccaaagag

SEQ ID NO: 19015 - RNA, 20 nt, synthetic construct
  source 1..20: mol_type = other RNA
agaggagcccaagccaaaga

SEQ ID NO: 19016 - RNA, 20 nt, synthetic construct
  source 1..20: mol_type = other RNA
cagaggagcccaagccaaag

SEQ ID NO: 19017 - RNA, 20 nt, synthetic construct
  source 1..20: mol_type = other RNA
cttgggctcctctggcatgc

SEQ ID NO: 19018 - RNA, 20 nt, synthetic construct
  source 1..20: mol_type = other RNA
ctcctctggcatgcaggaac

SEQ ID NO: 19019 - RNA, 20 nt, synthetic construct
  source 1..20: mol_type = other RNA
tcctctggcatgcaggaacc

SEQ ID NO: 19020 - RNA, 20 nt, synthetic construct
  source 1..20: mol_type = other RNA
tctggcatgcaggaaccggg

SEQ ID NO: 19021 - RNA, 20 nt, synthetic construct
  source 1..20: mol_type = other RNA
acccggttcctgcatgccag

SEQ ID NO: 19022 - RNA, 20 nt, synthetic construct
  source 1..20: mol_type = other RNA
aaccgggtggcatgagctct

SEQ ID NO: 19023 - RNA, 20 nt, synthetic construct
  source 1..20: mol_type = other RNA
accgggtggcatgagctcta

SEQ ID NO: 19024 - RNA, 20 nt, synthetic construct
  source 1..20: mol_type = other RNA
ccgggtggcatgagctctag

SEQ ID NO: 19025 - RNA, 20 nt, synthetic construct
  source 1..20: mol_type = other RNA
cccctagagctcatgccacc

SEQ ID NO: 19026 - RNA, 20 nt, synthetic construct
  source 1..20: mol_type = other RNA
atgagctctaggggtgaaga

SEQ ID NO: 19027 - RNA, 20 nt, synthetic construct
  source 1..20: mol_type = other RNA
agctctaggggtgaagaagg

SEQ ID NO: 19028 - RNA, 20 nt, synthetic construct
  source 1..20: mol_type = other RNA
gctctaggggtgaagaaggt

SEQ ID NO: 19029 - RNA, 20 nt, synthetic construct
  source 1..20: mol_type = other RNA
ctctaggggtgaagaaggtg

SEQ ID NO: 19030 - RNA, 20 nt, synthetic construct
  source 1..20: mol_type = other RNA
tcatcccgtgtgtcccgaag

SEQ ID NO: 19031 - RNA, 20 nt, synthetic construct
  source 1..20: mol_type = other RNA
catcccgtgtgtcccgaagt

SEQ ID NO: 19032 - RNA, 20 nt, synthetic construct
  source 1..20: mol_type = other RNA
atcccgtgtgtcccgaagtg

SEQ ID NO: 19033 - RNA, 20 nt, synthetic construct
  source 1..20: mol_type = other RNA
ggccccacttcgggacacac

SEQ ID NO: 19034 - RNA, 20 nt, synthetic construct
  source 1..20: mol_type = other RNA
tggccccacttcgggacaca

SEQ ID NO: 19035 - RNA, 20 nt, synthetic construct
  source 1..20: mol_type = other RNA
gaagtggggccagcacacac

SEQ ID NO: 19036 - RNA, 20 nt, synthetic construct
  source 1..20: mol_type = other RNA
aagtggggccagcacacaca

SEQ ID NO: 19037 - RNA, 20 nt, synthetic construct
  source 1..20: mol_type = other RNA
gtgtgtgctggccccacttc

SEQ ID NO: 19038 - RNA, 20 nt, synthetic construct
  source 1..20: mol_type = other RNA
tgtgtgtgctggccccactt

SEQ ID NO: 19039 - RNA, 20 nt, synthetic construct
  source 1..20: mol_type = other RNA
ctggggagccctgtgtgtgc

SEQ ID NO: 19040 - RNA, 20 nt, synthetic construct
  source 1..20: mol_type = other RNA
cagcccgagctacaaatccc

SEQ ID NO: 19041 - RNA, 20 nt, synthetic construct
  source 1..20: mol_type = other RNA
agcccgagctacaaatcccc

SEQ ID NO: 19042 - RNA, 20 nt, synthetic construct
  source 1..20: mol_type = other RNA
gggatttgtagctcgggctg

SEQ ID NO: 19043 - RNA, 20 nt, synthetic construct
  source 1..20: mol_type = other RNA
ggggatttgtagctcgggct

SEQ ID NO: 19044 - RNA, 20 nt, synthetic construct
  source 1..20: mol_type = other RNA
cggggatttgtagctcgggc

SEQ ID NO: 19045 - RNA, 20 nt, synthetic construct
  source 1..20: mol_type = other RNA
gtcccggggatttgtagctc

SEQ ID NO: 19046 - RNA, 20 nt, synthetic construct
  source 1..20: mol_type = other RNA
agtcccggggatttgtagct

SEQ ID NO: 19047 - RNA, 20 nt, synthetic construct
  source 1..20: mol_type = other RNA
caaatccccgggactgacct

SEQ ID NO: 19048 - RNA, 20 nt, synthetic construct
  source 1..20: mol_type = other RNA
cccgggactgaccttggtaa

SEQ ID NO: 19049 - RNA, 20 nt, synthetic construct
  source 1..20: mol_type = other RNA
cattaccaaggtcagtcccg

SEQ ID NO: 19050 - RNA, 20 nt, synthetic construct
  source 1..20: mol_type = other RNA
ccattaccaaggtcagtccc

SEQ ID NO: 19051 - RNA, 20 nt, synthetic construct
  source 1..20: mol_type = other RNA
tccattaccaaggtcagtcc

SEQ ID NO: 19052 - RNA, 20 nt, synthetic construct
  source 1..20: mol_type = other RNA
tgaccttggtaatggagcgg

SEQ ID NO: 19053 - RNA, 20 nt, synthetic construct
  source 1..20: mol_type = other RNA
gaccttggtaatggagcggc

SEQ ID NO: 19054 - RNA, 20 nt, synthetic construct
  source 1..20: mol_type = other RNA
gtcccgccgctccattacca

SEQ ID NO: 19055 - RNA, 20 nt, synthetic construct
  source 1..20: mol_type = other RNA
taatggagcggcgggacttg

SEQ ID NO: 19056 - RNA, 20 nt, synthetic construct
  source 1..20: mol_type = other RNA
gacttgcggctgcatctgat

SEQ ID NO: 19057 - RNA, 20 nt, synthetic construct
  source 1..20: mol_type = other RNA
acttgcggctgcatctgatc

SEQ ID NO: 19058 - RNA, 20 nt, synthetic construct
  source 1..20: mol_type = other RNA
gcggctgcatctgatcgggc

SEQ ID NO: 19059 - RNA, 20 nt, synthetic construct
  source 1..20: mol_type = other RNA
ctgcatctgatcgggcagga

SEQ ID NO: 19060 - RNA, 20 nt, synthetic construct
  source 1..20: mol_type = other RNA
atctgatcgggcaggaagga

SEQ ID NO: 19061 - RNA, 20 nt, synthetic construct
  source 1..20: mol_type = other RNA
tctgatcgggcaggaaggat

SEQ ID NO: 19062 - RNA, 20 nt, synthetic construct
  source 1..20: mol_type = other RNA
gggcaggaaggatgggtaat

SEQ ID NO: 19063 - RNA, 20 nt, synthetic construct
  source 1..20: mol_type = other RNA
ggcaggaaggatgggtaatt

SEQ ID NO: 19064 - RNA, 20 nt, synthetic construct
  source 1..20: mol_type = other RNA
aaggatgggtaattgggccc

SEQ ID NO: 19065 - RNA, 20 nt, synthetic construct
  source 1..20: mol_type = other RNA
aggatgggtaattgggcccc

SEQ ID NO: 19066 - RNA, 20 nt, synthetic construct
  source 1..20: mol_type = other RNA
atgggtaattgggccccggg

SEQ ID NO: 19067 - RNA, 20 nt, synthetic construct
  source 1..20: mol_type = other RNA
tgggtaattgggccccgggt

SEQ ID NO: 19068 - RNA, 20 nt, synthetic construct
  source 1..20: mol_type = other RNA
gggtaattgggccccgggtg

SEQ ID NO: 19069 - RNA, 20 nt, synthetic construct
  source 1..20: mol_type = other RNA
aattgggccccgggtgggga

SEQ ID NO: 19070 - RNA, 20 nt, synthetic construct
  source 1..20: mol_type = other RNA
ccccgggtggggatggaagc

SEQ ID NO: 19071 - RNA, 20 nt, synthetic construct
  source 1..20: mol_type = other RNA
cccgggtggggatggaagcc

SEQ ID NO: 19072 - RNA, 20 nt, synthetic construct
  source 1..20: mol_type = other RNA
gggtggggatggaagccggg

SEQ ID NO: 19073 - RNA, 20 nt, synthetic construct
  source 1..20: mol_type = other RNA
ccggcttccatccccacccg

SEQ ID NO: 19074 - RNA, 20 nt, synthetic construct
  source 1..20: mol_type = other RNA
cccggcttccatccccaccc

SEQ ID NO: 19075 - RNA, 20 nt, synthetic construct
  source 1..20: mol_type = other RNA
tcccggcttccatccccacc

SEQ ID NO: 19076 - RNA, 20 nt, synthetic construct
  source 1..20: mol_type = other RNA
ggatggaagccgggaggaag

SEQ ID NO: 19077 - RNA, 20 nt, synthetic construct
  source 1..20: mol_type = other RNA
ggaagccgggaggaagcggc

SEQ ID NO: 19078 - RNA, 20 nt, synthetic construct
  source 1..20: mol_type = other RNA
gaagccgggaggaagcggca

SEQ ID NO: 19079 - RNA, 20 nt, synthetic construct
  source 1..20: mol_type = other RNA
ccgggaggaagcggcagggc

SEQ ID NO: 19080 - RNA, 20 nt, synthetic construct
  source 1..20: mol_type = other RNA
cgggaggaagcggcagggca

SEQ ID NO: 19081 - RNA, 20 nt, synthetic construct
  source 1..20: mol_type = other RNA
cctgccctgccgcttcctcc

SEQ ID NO: 19082 - RNA, 20 nt, synthetic construct
  source 1..20: mol_type = other RNA
tgaggaagtgctgagcagca

SEQ ID NO: 19083 - RNA, 20 nt, synthetic construct
  source 1..20: mol_type = other RNA
ttgaggaagtgctgagcagc

SEQ ID NO: 19084 - RNA, 20 nt, synthetic construct
  source 1..20: mol_type = other RNA
tcagcacttcctcaagaccc

SEQ ID NO: 19085 - RNA, 20 nt, synthetic construct
  source 1..20: mol_type = other RNA
cagcacttcctcaagaccca

SEQ ID NO: 19086 - RNA, 20 nt, synthetic construct
  source 1..20: mol_type = other RNA
acttcctcaagacccagggt

SEQ ID NO: 19087 - RNA, 20 nt, synthetic construct
  source 1..20: mol_type = other RNA
cttcctcaagacccagggtc

SEQ ID NO: 19088 - RNA, 20 nt, synthetic construct
  source 1..20: mol_type = other RNA
ttcctcaagacccagggtcg

SEQ ID NO: 19089 - RNA, 20 nt, synthetic construct
  source 1..20: mol_type = other RNA
taccccgaccctgggtcttg

SEQ ID NO: 19090 - RNA, 20 nt, synthetic construct
  source 1..20: mol_type = other RNA
cagggtcggggtagtcctgc

SEQ ID NO: 19091 - RNA, 20 nt, synthetic construct
  source 1..20: mol_type = other RNA
agggtcggggtagtcctgct

SEQ ID NO: 19092 - RNA, 20 nt, synthetic construct
  source 1..20: mol_type = other RNA
gggtcggggtagtcctgctg

SEQ ID NO: 19093 - RNA, 20 nt, synthetic construct
  source 1..20: mol_type = other RNA
agcaggactaccccgaccct

SEQ ID NO: 19094 - RNA, 20 nt, synthetic construct
  source 1..20: mol_type = other RNA
cagcaggactaccccgaccc

SEQ ID NO: 19095 - RNA, 20 nt, synthetic construct
  source 1..20: mol_type = other RNA
tgctggggagctgccgcccc

SEQ ID NO: 19096 - RNA, 20 nt, synthetic construct
  source 1..20: mol_type = other RNA
gctggggagctgccgcccca

SEQ ID NO: 19097 - RNA, 20 nt, synthetic construct
  source 1..20: mol_type = other RNA
ctggggagctgccgccccag

SEQ ID NO: 19098 - RNA, 20 nt, synthetic construct
  source 1..20: mol_type = other RNA
tggggagctgccgccccagg

SEQ ID NO: 19099 - RNA, 20 nt, synthetic construct
  source 1..20: mol_type = other RNA
cacacgacttccccctgggg

SEQ ID NO: 19100 - RNA, 20 nt, synthetic construct
  source 1..20: mol_type = other RNA
agggggaagtcgtgtgcagc

SEQ ID NO: 19101 - RNA, 20 nt, synthetic construct
  source 1..20: mol_type = other RNA
ctgcacacgacttccccctg

SEQ ID NO: 19102 - RNA, 20 nt, synthetic construct
  source 1..20: mol_type = other RNA
gctgcacacgacttccccct

SEQ ID NO: 19103 - RNA, 20 nt, synthetic construct
  source 1..20: mol_type = other RNA
ggctgcacacgacttccccc

SEQ ID NO: 19104 - RNA, 20 nt, synthetic construct
  source 1..20: mol_type = other RNA
ggaagtcgtgtgcagccggc

SEQ ID NO: 19105 - RNA, 20 nt, synthetic construct
  source 1..20: mol_type = other RNA
agtcgtgtgcagccggccgg

SEQ ID NO: 19106 - RNA, 20 nt, synthetic construct
  source 1..20: mol_type = other RNA
ggccggtggccattgctgag

SEQ ID NO: 19107 - RNA, 20 nt, synthetic construct
  source 1..20: mol_type = other RNA
gccggtggccattgctgaga

SEQ ID NO: 19108 - RNA, 20 nt, synthetic construct
  source 1..20: mol_type = other RNA
ccggtggccattgctgagag

SEQ ID NO: 19109 - RNA, 20 nt, synthetic construct
  source 1..20: mol_type = other RNA
tctcagcaatggccaccggc

SEQ ID NO: 19110 - RNA, 20 nt, synthetic construct
  source 1..20: mol_type = other RNA
cccctctcagcaatggccac

SEQ ID NO: 19111 - RNA, 20 nt, synthetic construct
  source 1..20: mol_type = other RNA
gctggaccccctctcagcaa

SEQ ID NO: 19112 - RNA, 20 nt, synthetic construct
  source 1..20: mol_type = other RNA
gagggggtccagcgcccaag

SEQ ID NO: 19113 - RNA, 20 nt, synthetic construct
  source 1..20: mol_type = other RNA
agggggtccagcgcccaagt

SEQ ID NO: 19114 - RNA, 20 nt, synthetic construct
  source 1..20: mol_type = other RNA
tcgtgcacccacttgggcgc

SEQ ID NO: 19115 - RNA, 20 nt, synthetic construct
  source 1..20: mol_type = other RNA
gtctcttcgtgcacccactt

SEQ ID NO: 19116 - RNA, 20 nt, synthetic construct
  source 1..20: mol_type = other RNA
ggtctcttcgtgcacccact

SEQ ID NO: 19117 - RNA, 20 nt, synthetic construct
  source 1..20: mol_type = other RNA
gaccgcctcctgcttgatct

SEQ ID NO: 19118 - RNA, 20 nt, synthetic construct
  source 1..20: mol_type = other RNA
accgcctcctgcttgatctt

SEQ ID NO: 19119 - RNA, 20 nt, synthetic construct
  source 1..20: mol_type = other RNA
ccgcctcctgcttgatcttg

SEQ ID NO: 19120 - RNA, 20 nt, synthetic construct
  source 1..20: mol_type = other RNA
ccccaagatcaagcaggagg

SEQ ID NO: 19121 - RNA, 20 nt, synthetic construct
  source 1..20: mol_type = other RNA
gtgccccaagatcaagcagg

SEQ ID NO: 19122 - RNA, 20 nt, synthetic construct
  source 1..20: mol_type = other RNA
ttgatcttggggcacgtgcg

SEQ ID NO: 19123 - RNA, 20 nt, synthetic construct
  source 1..20: mol_type = other RNA
atcttggggcacgtgcgcgg

SEQ ID NO: 19124 - RNA, 20 nt, synthetic construct
  source 1..20: mol_type = other RNA
gcgcggcggcccgccgttgt

SEQ ID NO: 19125 - RNA, 20 nt, synthetic construct
  source 1..20: mol_type = other RNA
cgcggcggcccgccgttgta

SEQ ID NO: 19126 - RNA, 20 nt, synthetic construct
  source 1..20: mol_type = other RNA
tggtggcgccctacaacggc

SEQ ID NO: 19127 - RNA, 20 nt, synthetic construct
  source 1..20: mol_type = other RNA
gtggtggcgccctacaacgg

SEQ ID NO: 19128 - RNA, 20 nt, synthetic construct
  source 1..20: mol_type = other RNA
ttgtagggcgccaccaccac

SEQ ID NO: 19129 - RNA, 20 nt, synthetic construct
  source 1..20: mol_type = other RNA
tgtagggcgccaccaccacc

SEQ ID NO: 19130 - RNA, 20 nt, synthetic construct
  source 1..20: mol_type = other RNA
gtggtggtggcgccctacaa

SEQ ID NO: 19131 - RNA, 20 nt, synthetic construct
  source 1..20: mol_type = other RNA
agggcgccaccaccaccggg

SEQ ID NO: 19132 - RNA, 20 nt, synthetic construct
  source 1..20: mol_type = other RNA
cggcagccacccggtggtgg

SEQ ID NO: 19133 - RNA, 20 nt, synthetic construct
  source 1..20: mol_type = other RNA
ccaccgggtggctgccgtca

SEQ ID NO: 19134 - RNA, 20 nt, synthetic construct
  source 1..20: mol_type = other RNA
tgacggcagccacccggtgg

SEQ ID NO: 19135 - RNA, 20 nt, synthetic construct
  source 1..20: mol_type = other RNA
ccctgacggcagccacccgg

SEQ ID NO: 19136 - RNA, 20 nt, synthetic construct
  source 1..20: mol_type = other RNA
cagccctgacggcagccacc

SEQ ID NO: 19137 - RNA, 20 nt, synthetic construct
  source 1..20: mol_type = other RNA
gtcagcaaaggcagccctga

SEQ ID NO: 19138 - RNA, 20 nt, synthetic construct
  source 1..20: mol_type = other RNA
ttgctgacgctgatgaccga

SEQ ID NO: 19139 - RNA, 20 nt, synthetic construct
  source 1..20: mol_type = other RNA
tgctgacgctgatgaccgac

SEQ ID NO: 19140 - RNA, 20 nt, synthetic construct
  source 1..20: mol_type = other RNA
tcggtcatcagcgtcagcaa

SEQ ID NO: 19141 - RNA, 20 nt, synthetic construct
  source 1..20: mol_type = other RNA
cagcgagtacggcagcccgt

SEQ ID NO: 19142 - RNA, 20 nt, synthetic construct
  source 1..20: mol_type = other RNA
ggctgccgtactcgctgcca

SEQ ID NO: 19143 - RNA, 20 nt, synthetic construct
  source 1..20: mol_type = other RNA
gctgccgtactcgctgccag

SEQ ID NO: 19144 - RNA, 20 nt, synthetic construct
  source 1..20: mol_type = other RNA
agcgcccctggcagcgagta

SEQ ID NO: 19145 - RNA, 20 nt, synthetic construct
  source 1..20: mol_type = other RNA
aaggcgtcgctgagcgcccc

SEQ ID NO: 19146 - RNA, 20 nt, synthetic construct
  source 1..20: mol_type = other RNA
gatgggcaagttcgtgctga

SEQ ID NO: 19147 - RNA, 20 nt, synthetic construct
  source 1..20: mol_type = other RNA
ttgcccatcagcccgccacc

SEQ ID NO: 19148 - RNA, 20 nt, synthetic construct
  source 1..20: mol_type = other RNA
cccatcagcccgccacctgg

SEQ ID NO: 19149 - RNA, 20 nt, synthetic construct
  source 1..20: mol_type = other RNA
ccgccaggtggcgggctgat

SEQ ID NO: 19150 - RNA, 20 nt, synthetic construct
  source 1..20: mol_type = other RNA
agcccgccacctggcggctg

SEQ ID NO: 19151 - RNA, 20 nt, synthetic construct
  source 1..20: mol_type = other RNA
agccgcagccgccaggtggc

SEQ ID NO: 19152 - RNA, 20 nt, synthetic construct
  source 1..20: mol_type = other RNA
cagccgcagccgccaggtgg

SEQ ID NO: 19153 - RNA, 20 nt, synthetic construct
  source 1..20: mol_type = other RNA
cctggcggctgcggctgctg

SEQ ID NO: 19154 - RNA, 20 nt, synthetic construct
  source 1..20: mol_type = other RNA
cagcagccgcagccgccagg

SEQ ID NO: 19155 - RNA, 20 nt, synthetic construct
  source 1..20: mol_type = other RNA
ggcggctgcggctgctgcgg

SEQ ID NO: 19156 - RNA, 20 nt, synthetic construct
  source 1..20: mol_type = other RNA
ccgcagcagccgcagccgcc

SEQ ID NO: 19157 - RNA, 20 nt, synthetic construct
  source 1..20: mol_type = other RNA
tgctgcggcggaatgtacac

SEQ ID NO: 19158 - RNA, 20 nt, synthetic construct
  source 1..20: mol_type = other RNA
gctgcggcggaatgtacacc

SEQ ID NO: 19159 - RNA, 20 nt, synthetic construct
  source 1..20: mol_type = other RNA
atgtacaccgggtccaattc

SEQ ID NO: 19160 - RNA, 20 nt, synthetic construct
  source 1..20: mol_type = other RNA
ccgggtccaattctggccgc

SEQ ID NO: 19161 - RNA, 20 nt, synthetic construct
  source 1..20: mol_type = other RNA
cctgcggccagaattggacc

SEQ ID NO: 19162 - RNA, 20 nt, synthetic construct
  source 1..20: mol_type = other RNA
caattctggccgcaggagct

SEQ ID NO: 19163 - RNA, 20 nt, synthetic construct
  source 1..20: mol_type = other RNA
cgagctcctgcggccagaat

SEQ ID NO: 19164 - RNA, 20 nt, synthetic construct
  source 1..20: mol_type = other RNA
gcttcgtggccgagctcctg

SEQ ID NO: 19165 - RNA, 20 nt, synthetic construct
  source 1..20: mol_type = other RNA
ctcggccacgaagccgcccg

SEQ ID NO: 19166 - RNA, 20 nt, synthetic construct
  source 1..20: mol_type = other RNA
tcggccacgaagccgcccga

SEQ ID NO: 19167 - RNA, 20 nt, synthetic construct
  source 1..20: mol_type = other RNA
cggccacgaagccgcccgag

SEQ ID NO: 19168 - RNA, 20 nt, synthetic construct
  source 1..20: mol_type = other RNA
gagcccctcgggcggcttcg

SEQ ID NO: 19169 - RNA, 20 nt, synthetic construct
  source 1..20: mol_type = other RNA
aacgacgtgagcccctcggg

SEQ ID NO: 19170 - RNA, 20 nt, synthetic construct
  source 1..20: mol_type = other RNA
atcaacgacgtgagcccctc

SEQ ID NO: 19171 - RNA, 20 nt, synthetic construct
  source 1..20: mol_type = other RNA
catcaacgacgtgagcccct

SEQ ID NO: 19172 - RNA, 20 nt, synthetic construct
  source 1..20: mol_type = other RNA
tcacgtcgttgatgtccgcc

SEQ ID NO: 19173 - RNA, 20 nt, synthetic construct
  source 1..20: mol_type = other RNA
gttgatgtccgccaggttga

SEQ ID NO: 19174 - RNA, 20 nt, synthetic construct
  source 1..20: mol_type = other RNA
ttgatgtccgccaggttgaa

SEQ ID NO: 19175 - RNA, 20 nt, synthetic construct
  source 1..20: mol_type = other RNA
gccaggttgaagggagccgt

SEQ ID NO: 19176 - RNA, 20 nt, synthetic construct
  source 1..20: mol_type = other RNA
gacggctcccttcaacctgg

SEQ ID NO: 19177 - RNA, 20 nt, synthetic construct
  source 1..20: mol_type = other RNA
ggttgaagggagccgtcgga

SEQ ID NO: 19178 - RNA, 20 nt, synthetic construct
  source 1..20: mol_type = other RNA
gttgaagggagccgtcggag

SEQ ID NO: 19179 - RNA, 20 nt, synthetic construct
  source 1..20: mol_type = other RNA
ttgaagggagccgtcggagg

SEQ ID NO: 19180 - RNA, 20 nt, synthetic construct
  source 1..20: mol_type = other RNA
gggagccgtcggagggggag

SEQ ID NO: 19181 - RNA, 20 nt, synthetic construct
  source 1..20: mol_type = other RNA
ggagtccgctccccctccga

SEQ ID NO: 19182 - RNA, 20 nt, synthetic construct
  source 1..20: mol_type = other RNA
gagcggactccctgccatag

SEQ ID NO: 19183 - RNA, 20 nt, synthetic construct
  source 1..20: mol_type = other RNA
cggactccctgccatagagg

SEQ ID NO: 19184 - RNA, 20 nt, synthetic construct
  source 1..20: mol_type = other RNA
cggaggcctcctctatggca

SEQ ID NO: 19185 - RNA, 20 nt, synthetic construct
  source 1..20: mol_type = other RNA
gcggaggcctcctctatggc

SEQ ID NO: 19186 - RNA, 20 nt, synthetic construct
  source 1..20: mol_type = other RNA
acgggcggaggcctcctcta

SEQ ID NO: 19187 - RNA, 20 nt, synthetic construct
  source 1..20: mol_type = other RNA
aggcctccgcccgtgccgcc

SEQ ID NO: 19188 - RNA, 20 nt, synthetic construct
  source 1..20: mol_type = other RNA
gcgccgggcggcacgggcgg

SEQ ID NO: 19189 - RNA, 20 nt, synthetic construct
  source 1..20: mol_type = other RNA
gtggcgccgggcggcacggg

SEQ ID NO: 19190 - RNA, 20 nt, synthetic construct
  source 1..20: mol_type = other RNA
gtgccgcccggcgccacgcc

SEQ ID NO: 19191 - RNA, 20 nt, synthetic construct
  source 1..20: mol_type = other RNA
tgccgcccggcgccacgccc

SEQ ID NO: 19192 - RNA, 20 nt, synthetic construct
  source 1..20: mol_type = other RNA
ggcgtggcgccgggcggcac

SEQ ID NO: 19193 - RNA, 20 nt, synthetic construct
  source 1..20: mol_type = other RNA
gggcgtggcgccgggcggca

SEQ ID NO: 19194 - RNA, 20 nt, synthetic construct
  source 1..20: mol_type = other RNA
gacccgggcgtggcgccggg

SEQ ID NO: 19195 - RNA, 20 nt, synthetic construct
  source 1..20: mol_type = other RNA
cgccacgcccgggtcgttcc

SEQ ID NO: 19196 - RNA, 20 nt, synthetic construct
  source 1..20: mol_type = other RNA
gaacgacccgggcgtggcgc

SEQ ID NO: 19197 - RNA, 20 nt, synthetic construct
  source 1..20: mol_type = other RNA
cgcccgggtcgttcccggcc

SEQ ID NO: 19198 - RNA, 20 nt, synthetic construct
  source 1..20: mol_type = other RNA
ggccgggaacgacccgggcg

SEQ ID NO: 19199 - RNA, 20 nt, synthetic construct
  source 1..20: mol_type = other RNA
gggtcgttcccggcccggat

SEQ ID NO: 19200 - RNA, 20 nt, synthetic construct
  source 1..20: mol_type = other RNA
atccgggccgggaacgaccc

SEQ ID NO: 19201 - RNA, 20 nt, synthetic construct
  source 1..20: mol_type = other RNA
gatccgggccgggaacgacc

SEQ ID NO: 19202 - RNA, 20 nt, synthetic construct
  source 1..20: mol_type = other RNA
gttcccggcccggatcggat

SEQ ID NO: 19203 - RNA, 20 nt, synthetic construct
  source 1..20: mol_type = other RNA
tcacctatccgatccgggcc

SEQ ID NO: 19204 - RNA, 20 nt, synthetic construct
  source 1..20: mol_type = other RNA
ttcacctatccgatccgggc

SEQ ID NO: 19205 - RNA, 20 nt, synthetic construct
  source 1..20: mol_type = other RNA
gatcggataggtgaagctgc

SEQ ID NO: 19206 - RNA, 20 nt, synthetic construct
  source 1..20: mol_type = other RNA
cagcttcacctatccgatcc

SEQ ID NO: 19207 - RNA, 20 nt, synthetic construct
  source 1..20: mol_type = other RNA
gcagcttcacctatccgatc

SEQ ID NO: 19208 - RNA, 20 nt, synthetic construct
  source 1..20: mol_type = other RNA
cggataggtgaagctgcagg

SEQ ID NO: 19209 - RNA, 20 nt, synthetic construct
  source 1..20: mol_type = other RNA
ataggtgaagctgcaggtgg

SEQ ID NO: 19210 - RNA, 20 nt, synthetic construct
  source 1..20: mol_type = other RNA
taggtgaagctgcaggtgga

SEQ ID NO: 19211 - RNA, 20 nt, synthetic construct
  source 1..20: mol_type = other RNA
gctgcaggtggagggcgcgc

SEQ ID NO: 19212 - RNA, 20 nt, synthetic construct
  source 1..20: mol_type = other RNA
caggtggagggcgcgctggc

SEQ ID NO: 19213 - RNA, 20 nt, synthetic construct
  source 1..20: mol_type = other RNA
aggtggagggcgcgctggca

SEQ ID NO: 19214 - RNA, 20 nt, synthetic construct
  source 1..20: mol_type = other RNA
ctggcagggccgctgctcga

SEQ ID NO: 19215 - RNA, 20 nt, synthetic construct
  source 1..20: mol_type = other RNA
gctcgacggcgacgacgaag

SEQ ID NO: 19216 - RNA, 20 nt, synthetic construct
  source 1..20: mol_type = other RNA
cgacggcgacgacgaagagg

SEQ ID NO: 19217 - RNA, 20 nt, synthetic construct
  source 1..20: mol_type = other RNA
agaggaggctgacgctgacg

SEQ ID NO: 19218 - RNA, 20 nt, synthetic construct
  source 1..20: mol_type = other RNA
ggctgacgctgacgaggaca

SEQ ID NO: 19219 - RNA, 20 nt, synthetic construct
  source 1..20: mol_type = other RNA
tgacgctgacgaggacacgg

SEQ ID NO: 19220 - RNA, 20 nt, synthetic construct
  source 1..20: mol_type = other RNA
cgctgacgaggacacggtgg

SEQ ID NO: 19221 - RNA, 20 nt, synthetic construct
  source 1..20: mol_type = other RNA
acggtggcggccactgactc

SEQ ID NO: 19222 - RNA, 20 nt, synthetic construct
  source 1..20: mol_type = other RNA
gtggcggccactgactccgg

SEQ ID NO: 19223 - RNA, 20 nt, synthetic construct
  source 1..20: mol_type = other RNA
cggccactgactccggagga

SEQ ID NO: 19224 - RNA, 20 nt, synthetic construct
  source 1..20: mol_type = other RNA
ggccactgactccggaggat

SEQ ID NO: 19225 - RNA, 20 nt, synthetic construct
  source 1..20: mol_type = other RNA
gacccatcctccggagtcag

SEQ ID NO: 19226 - RNA, 20 nt, synthetic construct
  source 1..20: mol_type = other RNA
cggaggatgggtcagcgaat

SEQ ID NO: 19227 - RNA, 20 nt, synthetic construct
  source 1..20: mol_type = other RNA
caattcgctgacccatcctc

SEQ ID NO: 19228 - RNA, 20 nt, synthetic construct
  source 1..20: mol_type = other RNA
aattggagagaataaagtcc

SEQ ID NO: 19229 - RNA, 20 nt, synthetic construct
  source 1..20: mol_type = other RNA
agagaataaagtccaggtcc

SEQ ID NO: 19230 - RNA, 20 nt, synthetic construct
  source 1..20: mol_type = other RNA
gttcaacgatctcctggacc

SEQ ID NO: 19231 - RNA, 20 nt, synthetic construct
  source 1..20: mol_type = other RNA
caggagatcgttgaactcct

SEQ ID NO: 19232 - RNA, 20 nt, synthetic construct
  source 1..20: mol_type = other RNA
cgaggagttcaacgatctcc

SEQ ID NO: 19233 - RNA, 20 nt, synthetic construct
  source 1..20: mol_type = other RNA
aactcctcggtctctctccg

SEQ ID NO: 19234 - RNA, 20 nt, synthetic construct
  source 1..20: mol_type = other RNA
cctcggtctctctccgaggt

SEQ ID NO: 19235 - RNA, 20 nt, synthetic construct
  source 1..20: mol_type = other RNA
ctcggtctctctccgaggta

SEQ ID NO: 19236 - RNA, 20 nt, synthetic construct
  source 1..20: mol_type = other RNA
tcggtctctctccgaggtag

SEQ ID NO: 19237 - RNA, 20 nt, synthetic construct
  source 1..20: mol_type = other RNA
cctacctcggagagagaccg

SEQ ID NO: 19238 - RNA, 20 nt, synthetic construct
  source 1..20: mol_type = other RNA
ctctccgaggtaggggcgcc

SEQ ID NO: 19239 - RNA, 20 nt, synthetic construct
  source 1..20: mol_type = other RNA
gcaacctggcgcccctacct

SEQ ID NO: 19240 - RNA, 20 nt, synthetic construct
  source 1..20: mol_type = other RNA
ggcttgcggcggtagcaacc

SEQ ID NO: 19241 - RNA, 20 nt, synthetic construct
  source 1..20: mol_type = other RNA
gctaccgccgcaagccgcac

SEQ ID NO: 19242 - RNA, 20 nt, synthetic construct
  source 1..20: mol_type = other RNA
ggagccggtgcggcttgcgg

SEQ ID NO: 19243 - RNA, 20 nt, synthetic construct
  source 1..20: mol_type = other RNA
ggcggagccggtgcggcttg

SEQ ID NO: 19244 - RNA, 20 nt, synthetic construct
  source 1..20: mol_type = other RNA
caccggctccgccgctctcc

SEQ ID NO: 19245 - RNA, 20 nt, synthetic construct
  source 1..20: mol_type = other RNA
ggagagcggcggagccggtg

SEQ ID NO: 19246 - RNA, 20 nt, synthetic construct
  source 1..20: mol_type = other RNA
gacctggagagcggcggagc

SEQ ID NO: 19247 - RNA, 20 nt, synthetic construct
  source 1..20: mol_type = other RNA
gctctccaggtctgtggcca

SEQ ID NO: 19248 - RNA, 20 nt, synthetic construct
  source 1..20: mol_type = other RNA
gtggccacagacctggagag

SEQ ID NO: 19249 - RNA, 20 nt, synthetic construct
  source 1..20: mol_type = other RNA
ggcgaccgtggccacagacc

SEQ ID NO: 19250 - RNA, 20 nt, synthetic construct
  source 1..20: mol_type = other RNA
tggccacggtcgccgccgcc

SEQ ID NO: 19251 - RNA, 20 nt, synthetic construct
  source 1..20: mol_type = other RNA
ggtcgccgccgccaggtcat

SEQ ID NO: 19252 - RNA, 20 nt, synthetic construct
  source 1..20: mol_type = other RNA
tgacctggcggcggcgaccg

SEQ ID NO: 19253 - RNA, 20 nt, synthetic construct
  source 1..20: mol_type = other RNA
tcgccgccgccaggtcatag

SEQ ID NO: 19254 - RNA, 20 nt, synthetic construct
  source 1..20: mol_type = other RNA
ccgccgccaggtcatagggg

SEQ ID NO: 19255 - RNA, 20 nt, synthetic construct
  source 1..20: mol_type = other RNA
cgccaggtcataggggcggc

SEQ ID NO: 19256 - RNA, 20 nt, synthetic construct
  source 1..20: mol_type = other RNA
gccaggtcataggggcggcc

SEQ ID NO: 19257 - RNA, 20 nt, synthetic construct
  source 1..20: mol_type = other RNA
cggccgcccctatgacctgg

SEQ ID NO: 19258 - RNA, 20 nt, synthetic construct
  source 1..20: mol_type = other RNA
tcccggccgcccctatgacc

SEQ ID NO: 19259 - RNA, 20 nt, synthetic construct
  source 1..20: mol_type = other RNA
taggggcggccgggaagcac

SEQ ID NO: 19260 - RNA, 20 nt, synthetic construct
  source 1..20: mol_type = other RNA
aggggcggccgggaagcact

SEQ ID NO: 19261 - RNA, 20 nt, synthetic construct
  source 1..20: mol_type = other RNA
ggggcggccgggaagcactg

SEQ ID NO: 19262 - RNA, 20 nt, synthetic construct
  source 1..20: mol_type = other RNA
gggcggccgggaagcactgg

SEQ ID NO: 19263 - RNA, 20 nt, synthetic construct
  source 1..20: mol_type = other RNA
cgacttcccccagtgcttcc

SEQ ID NO: 19264 - RNA, 20 nt, synthetic construct
  source 1..20: mol_type = other RNA
ctgggggaagtcgcttcatg

SEQ ID NO: 19265 - RNA, 20 nt, synthetic construct
  source 1..20: mol_type = other RNA
tgggggaagtcgcttcatgt

SEQ ID NO: 19266 - RNA, 20 nt, synthetic construct
  source 1..20: mol_type = other RNA
agctcctcccgccagcgctg

SEQ ID NO: 19267 - RNA, 20 nt, synthetic construct
  source 1..20: mol_type = other RNA
gctcctcccgccagcgctgc

SEQ ID NO: 19268 - RNA, 20 nt, synthetic construct
  source 1..20: mol_type = other RNA
ctcctcccgccagcgctgcg

SEQ ID NO: 19269 - RNA, 20 nt, synthetic construct
  source 1..20: mol_type = other RNA
cccgccagcgctgcggggac

SEQ ID NO: 19270 - RNA, 20 nt, synthetic construct
  source 1..20: mol_type = other RNA
ccgccagcgctgcggggaca

SEQ ID NO: 19271 - RNA, 20 nt, synthetic construct
  source 1..20: mol_type = other RNA
gtccccgcagcgctggcggg

SEQ ID NO: 19272 - RNA, 20 nt, synthetic construct
  source 1..20: mol_type = other RNA
ccagcgctgcggggacaggg

SEQ ID NO: 19273 - RNA, 20 nt, synthetic construct
  source 1..20: mol_type = other RNA
cagcgctgcggggacagggc

SEQ ID NO: 19274 - RNA, 20 nt, synthetic construct
  source 1..20: mol_type = other RNA
ccctgtccccgcagcgctgg

SEQ ID NO: 19275 - RNA, 20 nt, synthetic construct
  source 1..20: mol_type = other RNA
ccgccctgtccccgcagcgc

SEQ ID NO: 19276 - RNA, 20 nt, synthetic construct
  source 1..20: mol_type = other RNA
gggcgggagagacctgtcag

SEQ ID NO: 19277 - RNA, 20 nt, synthetic construct
  source 1..20: mol_type = other RNA
cgggagagacctgtcagtgg

SEQ ID NO: 19278 - RNA, 20 nt, synthetic construct
  source 1..20: mol_type = other RNA
aacaggggaccaccactgac

SEQ ID NO: 19279 - RNA, 20 nt, synthetic construct
  source 1..20: mol_type = other RNA
agtatgtcgggtggcaacag

SEQ ID NO: 19280 - RNA, 20 nt, synthetic construct
  source 1..20: mol_type = other RNA
cagtatgtcgggtggcaaca

SEQ ID NO: 19281 - RNA, 20 nt, synthetic construct
  source 1..20: mol_type = other RNA
tcagtatgtcgggtggcaac

SEQ ID NO: 19282 - RNA, 20 nt, synthetic construct
  source 1..20: mol_type = other RNA
cacccgacatactgacgtgc

SEQ ID NO: 19283 - RNA, 20 nt, synthetic construct
  source 1..20: mol_type = other RNA
ccgacatactgacgtgctgg

SEQ ID NO: 19284 - RNA, 20 nt, synthetic construct
  source 1..20: mol_type = other RNA
cagcacgtcagtatgtcggg

SEQ ID NO: 19285 - RNA, 20 nt, synthetic construct
  source 1..20: mol_type = other RNA
cgccagcacgtcagtatgtc

SEQ ID NO: 19286 - RNA, 20 nt, synthetic construct
  source 1..20: mol_type = other RNA
ccgccagcacgtcagtatgt

SEQ ID NO: 19287 - RNA, 20 nt, synthetic construct
  source 1..20: mol_type = other RNA
ctgggcggtgcagtcgcgcg

SEQ ID NO: 19288 - RNA, 20 nt, synthetic construct
  source 1..20: mol_type = other RNA
gcgactgcaccgcccagaca

SEQ ID NO: 19289 - RNA, 20 nt, synthetic construct
  source 1..20: mol_type = other RNA
cgactgcaccgcccagacat

SEQ ID NO: 19290 - RNA, 20 nt, synthetic construct
  source 1..20: mol_type = other RNA
gactgcaccgcccagacatg

SEQ ID NO: 19291 - RNA, 20 nt, synthetic construct
  source 1..20: mol_type = other RNA
caccgcccagacatggggac

SEQ ID NO: 19292 - RNA, 20 nt, synthetic construct
  source 1..20: mol_type = other RNA
cccagacatggggactggtc

SEQ ID NO: 19293 - RNA, 20 nt, synthetic construct
  source 1..20: mol_type = other RNA
gaccagtccccatgtctggg

SEQ ID NO: 19294 - RNA, 20 nt, synthetic construct
  source 1..20: mol_type = other RNA
gacatggggactggtcaggc

SEQ ID NO: 19295 - RNA, 20 nt, synthetic construct
  source 1..20: mol_type = other RNA
cctgaccagtccccatgtct

SEQ ID NO: 19296 - RNA, 20 nt, synthetic construct
  source 1..20: mol_type = other RNA
gcctgaccagtccccatgtc

SEQ ID NO: 19297 - RNA, 20 nt, synthetic construct
  source 1..20: mol_type = other RNA
ggtaaggagcggccaccgcg

SEQ ID NO: 19298 - RNA, 20 nt, synthetic construct
  source 1..20: mol_type = other RNA
cgctccttaccctcgttcag

SEQ ID NO: 19299 - RNA, 20 nt, synthetic construct
  source 1..20: mol_type = other RNA
cactgaacgagggtaaggag

SEQ ID NO: 19300 - RNA, 20 nt, synthetic construct
  source 1..20: mol_type = other RNA
taccctcgttcagtggctct

SEQ ID NO: 19301 - RNA, 20 nt, synthetic construct
  source 1..20: mol_type = other RNA
agagccactgaacgagggta

SEQ ID NO: 19302 - RNA, 20 nt, synthetic construct
  source 1..20: mol_type = other RNA
caccaagagccactgaacga

SEQ ID NO: 19303 - RNA, 20 nt, synthetic construct
  source 1..20: mol_type = other RNA
tcaccaagagccactgaacg

SEQ ID NO: 19304 - RNA, 20 nt, synthetic construct
  source 1..20: mol_type = other RNA
agtggctcttggtgacccca

SEQ ID NO: 19305 - RNA, 20 nt, synthetic construct
  source 1..20: mol_type = other RNA
tgggggcgggcggagccttg

SEQ ID NO: 19306 - RNA, 20 nt, synthetic construct
  source 1..20: mol_type = other RNA
gtgggggcgggcggagcctt

SEQ ID NO: 19307 - RNA, 20 nt, synthetic construct
  source 1..20: mol_type = other RNA
ggtgggggcgggcggagcct

SEQ ID NO: 19308 - RNA, 20 nt, synthetic construct
  source 1..20: mol_type = other RNA
gtgggtgtggtgggggcggg

SEQ ID NO: 19309 - RNA, 20 nt, synthetic construct
  source 1..20: mol_type = other RNA
ttcgtgggtgtggtgggggc

SEQ ID NO: 19310 - RNA, 20 nt, synthetic construct
  source 1..20: mol_type = other RNA
tttcgtgggtgtggtggggg

SEQ ID NO: 19311 - RNA, 20 nt, synthetic construct
  source 1..20: mol_type = other RNA
ggttttcgtgggtgtggtgg

SEQ ID NO: 19312 - RNA, 20 nt, synthetic construct
  source 1..20: mol_type = other RNA
ccacacccacgaaaacccac

SEQ ID NO: 19313 - RNA, 20 nt, synthetic construct
  source 1..20: mol_type = other RNA
cacacccacgaaaacccacc

SEQ ID NO: 19314 - RNA, 20 nt, synthetic construct
  source 1..20: mol_type = other RNA
gtgggttttcgtgggtgtgg

SEQ ID NO: 19315 - RNA, 20 nt, synthetic construct
  source 1..20: mol_type = other RNA
ccggtgggttttcgtgggtg

SEQ ID NO: 19316 - RNA, 20 nt, synthetic construct
  source 1..20: mol_type = other RNA
gaaaacccaccgggcgttcc

SEQ ID NO: 19317 - RNA, 20 nt, synthetic construct
  source 1..20: mol_type = other RNA
gaacgcccggtgggttttcg

SEQ ID NO: 19318 - RNA, 20 nt, synthetic construct
  source 1..20: mol_type = other RNA
aacccaccgggcgttcccgg

SEQ ID NO: 19319 - RNA, 20 nt, synthetic construct
  source 1..20: mol_type = other RNA
accgggcgttcccggcggcc

SEQ ID NO: 19320 - RNA, 20 nt, synthetic construct
  source 1..20: mol_type = other RNA
ggccgccgggaacgcccggt

SEQ ID NO: 19321 - RNA, 20 nt, synthetic construct
  source 1..20: mol_type = other RNA
gggccgccgggaacgcccgg

SEQ ID NO: 19322 - RNA, 20 nt, synthetic construct
  source 1..20: mol_type = other RNA
tccgggccgccgggaacgcc

SEQ ID NO: 19323 - RNA, 20 nt, synthetic construct
  source 1..20: mol_type = other RNA
gagtatcgctccgggccgcc

SEQ ID NO: 19324 - RNA, 20 nt, synthetic construct
  source 1..20: mol_type = other RNA
tgagtatcgctccgggccgc

SEQ ID NO: 19325 - RNA, 20 nt, synthetic construct
  source 1..20: mol_type = other RNA
ggagcgatactcacgttatt

SEQ ID NO: 19326 - RNA, 20 nt, synthetic construct
  source 1..20: mol_type = other RNA
gagcgatactcacgttattc

SEQ ID NO: 19327 - RNA, 20 nt, synthetic construct
  source 1..20: mol_type = other RNA
aataacgtgagtatcgctcc

SEQ ID NO: 19328 - RNA, 20 nt, synthetic construct
  source 1..20: mol_type = other RNA
gaataacgtgagtatcgctc

SEQ ID NO: 19329 - RNA, 20 nt, synthetic construct
  source 1..20: mol_type = other RNA
gagaagacactgcgtcaagc

SEQ ID NO: 19330 - RNA, 20 nt, synthetic construct
  source 1..20: mol_type = other RNA
agtgtcttctcccttcccgc

SEQ ID NO: 19331 - RNA, 20 nt, synthetic construct
  source 1..20: mol_type = other RNA
gtgtcttctcccttcccgcc

SEQ ID NO: 19332 - RNA, 20 nt, synthetic construct
  source 1..20: mol_type = other RNA
cgcgtctggcccggcgggaa

SEQ ID NO: 19333 - RNA, 20 nt, synthetic construct
  source 1..20: mol_type = other RNA
tcgcgtctggcccggcggga

SEQ ID NO: 19334 - RNA, 20 nt, synthetic construct
  source 1..20: mol_type = other RNA
cgccgggccagacgcgaacg

SEQ ID NO: 19335 - RNA, 20 nt, synthetic construct
  source 1..20: mol_type = other RNA
acgttcgcgtctggcccggc

SEQ ID NO: 19336 - RNA, 20 nt, synthetic construct
  source 1..20: mol_type = other RNA
cacgttcgcgtctggcccgg

SEQ ID NO: 19337 - RNA, 20 nt, synthetic construct
  source 1..20: mol_type = other RNA
ctccacgttcgcgtctggcc

SEQ ID NO: 19338 - RNA, 20 nt, synthetic construct
  source 1..20: mol_type = other RNA
gacgcgaacgtggagaaaga

SEQ ID NO: 19339 - RNA, 20 nt, synthetic construct
  source 1..20: mol_type = other RNA
acgcgaacgtggagaaagat

SEQ ID NO: 19340 - RNA, 20 nt, synthetic construct
  source 1..20: mol_type = other RNA
tctttctccacgttcgcgtc

SEQ ID NO: 19341 - RNA, 20 nt, synthetic construct
  source 1..20: mol_type = other RNA
acagccatgtcagactcgcc

SEQ ID NO: 19342 - RNA, 20 nt, synthetic construct
  source 1..20: mol_type = other RNA
gccatgtcagactcgccagg

SEQ ID NO: 19343 - RNA, 20 nt, synthetic construct
  source 1..20: mol_type = other RNA
gccacctggcgagtctgaca

SEQ ID NO: 19344 - RNA, 20 nt, synthetic construct
  source 1..20: mol_type = other RNA
caggtggctgcctgcgagca

SEQ ID NO: 19345 - RNA, 20 nt, synthetic construct
  source 1..20: mol_type = other RNA
cttgctcgcaggcagccacc

SEQ ID NO: 19346 - RNA, 20 nt, synthetic construct
  source 1..20: mol_type = other RNA
ggctgcctgcgagcaaggca

SEQ ID NO: 19347 - RNA, 20 nt, synthetic construct
  source 1..20: mol_type = other RNA
cctgcgagcaaggcagggag

SEQ ID NO: 19348 - RNA, 20 nt, synthetic construct
  source 1..20: mol_type = other RNA
ccgctccctgccttgctcgc

SEQ ID NO: 19349 - RNA, 20 nt, synthetic construct
  source 1..20: mol_type = other RNA
gcaaggcagggagcggagac

SEQ ID NO: 19350 - RNA, 20 nt, synthetic construct
  source 1..20: mol_type = other RNA
ggagcggagacaggagagtc

SEQ ID NO: 19351 - RNA, 20 nt, synthetic construct
  source 1..20: mol_type = other RNA
gagcggagacaggagagtca

SEQ ID NO: 19352 - RNA, 20 nt, synthetic construct
  source 1..20: mol_type = other RNA
agcggagacaggagagtcag

SEQ ID NO: 19353 - RNA, 20 nt, synthetic construct
  source 1..20: mol_type = other RNA
ggagacaggagagtcagggg

SEQ ID NO: 19354 - RNA, 20 nt, synthetic construct
  source 1..20: mol_type = other RNA
ggagagtcaggggcggcttt

SEQ ID NO: 19355 - RNA, 20 nt, synthetic construct
  source 1..20: mol_type = other RNA
gcggctttcggccgtcgttc

SEQ ID NO: 19356 - RNA, 20 nt, synthetic construct
  source 1..20: mol_type = other RNA
gtcgttccggcgcgtcccac

SEQ ID NO: 19357 - RNA, 20 nt, synthetic construct
  source 1..20: mol_type = other RNA
ggtgggacgcgccggaacga

SEQ ID NO: 19358 - RNA, 20 nt, synthetic construct
  source 1..20: mol_type = other RNA
tgaggaccggtgggacgcgc

SEQ ID NO: 19359 - RNA, 20 nt, synthetic construct
  source 1..20: mol_type = other RNA
agggaggggtgaggaccggt

SEQ ID NO: 19360 - RNA, 20 nt, synthetic construct
  source 1..20: mol_type = other RNA
cagggaggggtgaggaccgg

SEQ ID NO: 19361 - RNA, 20 nt, synthetic construct
  source 1..20: mol_type = other RNA
gagcagggaggggtgaggac

SEQ ID NO: 19362 - RNA, 20 nt, synthetic construct
  source 1..20: mol_type = other RNA
gctgggagcagggaggggtg

SEQ ID NO: 19363 - RNA, 20 nt, synthetic construct
  source 1..20: mol_type = other RNA
gcggcgctgggagcagggag

SEQ ID NO: 19364 - RNA, 20 nt, synthetic construct
  source 1..20: mol_type = other RNA
cgcggcgctgggagcaggga

SEQ ID NO: 19365 - RNA, 20 nt, synthetic construct
  source 1..20: mol_type = other RNA
gcgcggcgctgggagcaggg

SEQ ID NO: 19366 - RNA, 20 nt, synthetic construct
  source 1..20: mol_type = other RNA
ggcgcgcggcgctgggagca

SEQ ID NO: 19367 - RNA, 20 nt, synthetic construct
  source 1..20: mol_type = other RNA
aggcgcgcggcgctgggagc

SEQ ID NO: 19368 - RNA, 20 nt, synthetic construct
  source 1..20: mol_type = other RNA
taggtgaggcgcgcggcgct

SEQ ID NO: 19369 - RNA, 20 nt, synthetic construct
  source 1..20: mol_type = other RNA
gtaggtgaggcgcgcggcgc

SEQ ID NO: 19370 - RNA, 20 nt, synthetic construct
  source 1..20: mol_type = other RNA
aatgaggtaggtgaggcgcg

SEQ ID NO: 19371 - RNA, 20 nt, synthetic construct
  source 1..20: mol_type = other RNA
cctcacctacctcattaatg

SEQ ID NO: 19372 - RNA, 20 nt, synthetic construct
  source 1..20: mol_type = other RNA
ctcacctacctcattaatgt

SEQ ID NO: 19373 - RNA, 20 nt, synthetic construct
  source 1..20: mol_type = other RNA
tcacctacctcattaatgtg

SEQ ID NO: 19374 - RNA, 20 nt, synthetic construct
  source 1..20: mol_type = other RNA
cacctacctcattaatgtgg

SEQ ID NO: 19375 - RNA, 20 nt, synthetic construct
  source 1..20: mol_type = other RNA
ccacattaatgaggtaggtg

SEQ ID NO: 19376 - RNA, 20 nt, synthetic construct
  source 1..20: mol_type = other RNA
ggcccccacattaatgaggt

SEQ ID NO: 19377 - RNA, 20 nt, synthetic construct
  source 1..20: mol_type = other RNA
cattaatgtgggggcccaga

SEQ ID NO: 19378 - RNA, 20 nt, synthetic construct
  source 1..20: mol_type = other RNA
tctgggcccccacattaatg

SEQ ID NO: 19379 - RNA, 20 nt, synthetic construct
  source 1..20: mol_type = other RNA
gtgggggcccagaaggtcct

SEQ ID NO: 19380 - RNA, 20 nt, synthetic construct
  source 1..20: mol_type = other RNA
cgggctgccgaggaccttct

SEQ ID NO: 19381 - RNA, 20 nt, synthetic construct
  source 1..20: mol_type = other RNA
tcgggctgccgaggaccttc

SEQ ID NO: 19382 - RNA, 20 nt, synthetic construct
  source 1..20: mol_type = other RNA
cctcggcagcccgaagcagc

SEQ ID NO: 19383 - RNA, 20 nt, synthetic construct
  source 1..20: mol_type = other RNA
ctcggcagcccgaagcagct

SEQ ID NO: 19384 - RNA, 20 nt, synthetic construct
  source 1..20: mol_type = other RNA
tcggcagcccgaagcagctg

SEQ ID NO: 19385 - RNA, 20 nt, synthetic construct
  source 1..20: mol_type = other RNA
ccagctgcttcgggctgccg

SEQ ID NO: 19386 - RNA, 20 nt, synthetic construct
  source 1..20: mol_type = other RNA
tcaggtgccccagctgcttc

SEQ ID NO: 19387 - RNA, 20 nt, synthetic construct
  source 1..20: mol_type = other RNA
ttcaggtgccccagctgctt

SEQ ID NO: 19388 - RNA, 20 nt, synthetic construct
  source 1..20: mol_type = other RNA
cttcgttgactttggggttc

SEQ ID NO: 19389 - RNA, 20 nt, synthetic construct
  source 1..20: mol_type = other RNA
tcttctcttcgttgactttg

SEQ ID NO: 19390 - RNA, 20 nt, synthetic construct
  source 1..20: mol_type = other RNA
ttcttctcttcgttgacttt

SEQ ID NO: 19391 - RNA, 20 nt, synthetic construct
  source 1..20: mol_type = other RNA
tttcttctcttcgttgactt

SEQ ID NO: 19392 - RNA, 20 nt, synthetic construct
  source 1..20: mol_type = other RNA
caaaacccaaaaccccaaat

SEQ ID NO: 19393 - RNA, 20 nt, synthetic construct
  source 1..20: mol_type = other RNA
caatttggggttttgggttt

SEQ ID NO: 19394 - RNA, 20 nt, synthetic construct
  source 1..20: mol_type = other RNA
ctcggccaatttggggtttt

SEQ ID NO: 19395 - RNA, 20 nt, synthetic construct
  source 1..20: mol_type = other RNA
tctcggccaatttggggttt

SEQ ID NO: 19396 - RNA, 20 nt, synthetic construct
  source 1..20: mol_type = other RNA
gaaggatctcggccaatttg

SEQ ID NO: 19397 - RNA, 20 nt, synthetic construct
  source 1..20: mol_type = other RNA
agaaggatctcggccaattt

SEQ ID NO: 19398 - RNA, 20 nt, synthetic construct
  source 1..20: mol_type = other RNA
aagaaggatctcggccaatt

SEQ ID NO: 19399 - RNA, 20 nt, synthetic construct
  source 1..20: mol_type = other RNA
tggccgagatccttcttctt

SEQ ID NO: 19400 - RNA, 20 nt, synthetic construct
  source 1..20: mol_type = other RNA
aatccaaagaagaaggatct

SEQ ID NO: 19401 - RNA, 20 nt, synthetic construct
  source 1..20: mol_type = other RNA
tatatttaatccaaagaaga

SEQ ID NO: 19402 - RNA, 20 nt, synthetic construct
  source 1..20: mol_type = other RNA
tctttggattaaatataact

SEQ ID NO: 19403 - RNA, 20 nt, synthetic construct
  source 1..20: mol_type = other RNA
ctaagaacttttgtatacaa

SEQ ID NO: 19404 - RNA, 20 nt, synthetic construct
  source 1..20: mol_type = other RNA
gcaaaaatagacaatcagca

SEQ ID NO: 19405 - RNA, 20 nt, synthetic construct
  source 1..20: mol_type = other RNA
aatcagcaaggcgagtaagt

SEQ ID NO: 19406 - RNA, 20 nt, synthetic construct
  source 1..20: mol_type = other RNA
gcaaggcgagtaagtaggtc

SEQ ID NO: 19407 - RNA, 20 nt, synthetic construct
  source 1..20: mol_type = other RNA
aggcgagtaagtaggtccgg

SEQ ID NO: 19408 - RNA, 20 nt, synthetic construct
  source 1..20: mol_type = other RNA
gagtaagtaggtccggtggc

SEQ ID NO: 19409 - RNA, 20 nt, synthetic construct
  source 1..20: mol_type = other RNA
agtaagtaggtccggtggcc

SEQ ID NO: 19410 - RNA, 20 nt, synthetic construct
  source 1..20: mol_type = other RNA
agagagcgcagcccggccac

SEQ ID NO: 19411 - RNA, 20 nt, synthetic construct
  source 1..20: mol_type = other RNA
gagtggaagagagcgcagcc

SEQ ID NO: 19412 - RNA, 20 nt, synthetic construct
  source 1..20: mol_type = other RNA
tggtgggggacgctgctgag

SEQ ID NO: 19413 - RNA, 20 nt, synthetic construct
  source 1..20: mol_type = other RNA
agcgtcccccaccactgtcg

SEQ ID NO: 19414 - RNA, 20 nt, synthetic construct
  source 1..20: mol_type = other RNA
ggcgaccgcgacagtggtgg

SEQ ID NO: 19415 - RNA, 20 nt, synthetic construct
  source 1..20: mol_type = other RNA
aggcgaccgcgacagtggtg

SEQ ID NO: 19416 - RNA, 20 nt, synthetic construct
  source 1..20: mol_type = other RNA
gaggcgaccgcgacagtggt

SEQ ID NO: 19417 - RNA, 20 nt, synthetic construct
  source 1..20: mol_type = other RNA
cgaggcgaccgcgacagtgg

SEQ ID NO: 19418 - RNA, 20 nt, synthetic construct
  source 1..20: mol_type = other RNA
actcgaggcgaccgcgacag

SEQ ID NO: 19419 - RNA, 20 nt, synthetic construct
  source 1..20: mol_type = other RNA
ggtcgcctcgagtgctgccg

SEQ ID NO: 19420 - RNA, 20 nt, synthetic construct
  source 1..20: mol_type = other RNA
gtcgcctcgagtgctgccgt

SEQ ID NO: 19421 - RNA, 20 nt, synthetic construct
  source 1..20: mol_type = other RNA
tcgagtgctgccgtgggcgc

SEQ ID NO: 19422 - RNA, 20 nt, synthetic construct
  source 1..20: mol_type = other RNA
cgagtgctgccgtgggcgca

SEQ ID NO: 19423 - RNA, 20 nt, synthetic construct
  source 1..20: mol_type = other RNA
gagtgctgccgtgggcgcag

SEQ ID NO: 19424 - RNA, 20 nt, synthetic construct
  source 1..20: mol_type = other RNA
tgcgcccacggcagcactcg

SEQ ID NO: 19425 - RNA, 20 nt, synthetic construct
  source 1..20: mol_type = other RNA
tgccgtgggcgcaggggctg

SEQ ID NO: 19426 - RNA, 20 nt, synthetic construct
  source 1..20: mol_type = other RNA
gtgggcgcaggggctgtggc

SEQ ID NO: 19427 - RNA, 20 nt, synthetic construct
  source 1..20: mol_type = other RNA
tgggcgcaggggctgtggcc

SEQ ID NO: 19428 - RNA, 20 nt, synthetic construct
  source 1..20: mol_type = other RNA
gggcgcaggggctgtggccg

SEQ ID NO: 19429 - RNA, 20 nt, synthetic construct
  source 1..20: mol_type = other RNA
ggccacagcccctgcgccca

SEQ ID NO: 19430 - RNA, 20 nt, synthetic construct
  source 1..20: mol_type = other RNA
cgcaggggctgtggccgggg

SEQ ID NO: 19431 - RNA, 20 nt, synthetic construct
  source 1..20: mol_type = other RNA
aggggctgtggccggggcgg

SEQ ID NO: 19432 - RNA, 20 nt, synthetic construct
  source 1..20: mol_type = other RNA
ggggctgtggccggggcggt

SEQ ID NO: 19433 - RNA, 20 nt, synthetic construct
  source 1..20: mol_type = other RNA
gctgtggccggggcggtggg

SEQ ID NO: 19434 - RNA, 20 nt, synthetic construct
  source 1..20: mol_type = other RNA
ctgtggccggggcggtgggc

SEQ ID NO: 19435 - RNA, 20 nt, synthetic construct
  source 1..20: mol_type = other RNA
tggccggggcggtgggcggg

SEQ ID NO: 19436 - RNA, 20 nt, synthetic construct
  source 1..20: mol_type = other RNA
gcaccgcccgcccaccgccc

SEQ ID NO: 19437 - RNA, 20 nt, synthetic construct
  source 1..20: mol_type = other RNA
ggtgggcgggcggtgccgcc

SEQ ID NO: 19438 - RNA, 20 nt, synthetic construct
  source 1..20: mol_type = other RNA
gcggtgccgccaggtgagac

SEQ ID NO: 19439 - RNA, 20 nt, synthetic construct
  source 1..20: mol_type = other RNA
ccaggtgagactggctgccg

SEQ ID NO: 19440 - RNA, 20 nt, synthetic construct
  source 1..20: mol_type = other RNA
cggcagccagtctcacctgg

SEQ ID NO: 19441 - RNA, 20 nt, synthetic construct
  source 1..20: mol_type = other RNA
ccacggcagccagtctcacc

SEQ ID NO: 19442 - RNA, 20 nt, synthetic construct
  source 1..20: mol_type = other RNA
cgtggcgcggagctgcgaac

SEQ ID NO: 19443 - RNA, 20 nt, synthetic construct
  source 1..20: mol_type = other RNA
cagttcgcagctccgcgcca

SEQ ID NO: 19444 - RNA, 20 nt, synthetic construct
  source 1..20: mol_type = other RNA
cggagctgcgaactggtcgg

SEQ ID NO: 19445 - RNA, 20 nt, synthetic construct
  source 1..20: mol_type = other RNA
gcgaactggtcggcggcgca

SEQ ID NO: 19446 - RNA, 20 nt, synthetic construct
  source 1..20: mol_type = other RNA
ctggtcggcggcgcaaggcg

SEQ ID NO: 19447 - RNA, 20 nt, synthetic construct
  source 1..20: mol_type = other RNA
gcggcgcaaggcgcggactc

SEQ ID NO: 19448 - RNA, 20 nt, synthetic construct
  source 1..20: mol_type = other RNA
gcggactccggtgagttgtg

SEQ ID NO: 19449 - RNA, 20 nt, synthetic construct
  source 1..20: mol_type = other RNA
tgagttgtgtggagcgcgcg

SEQ ID NO: 19450 - RNA, 20 nt, synthetic construct
  source 1..20: mol_type = other RNA
gcgcgctccacacaactcac

SEQ ID NO: 19451 - RNA, 20 nt, synthetic construct
  source 1..20: mol_type = other RNA
gtgtggagcgcgcgcggcca

SEQ ID NO: 19452 - RNA, 20 nt, synthetic construct
  source 1..20: mol_type = other RNA
tgtggagcgcgcgcggccat

SEQ ID NO: 19453 - RNA, 20 nt, synthetic construct
  source 1..20: mol_type = other RNA
agcgcgcgcggccatgggcg

SEQ ID NO: 19454 - RNA, 20 nt, synthetic construct
  source 1..20: mol_type = other RNA
gcgcgcgcggccatgggcgc

SEQ ID NO: 19455 - RNA, 20 nt, synthetic construct
  source 1..20: mol_type = other RNA
gcggccatgggcgcgggcca

SEQ ID NO: 19456 - RNA, 20 nt, synthetic construct
  source 1..20: mol_type = other RNA
cggccatgggcgcgggccac

SEQ ID NO: 19457 - RNA, 20 nt, synthetic construct
  source 1..20: mol_type = other RNA
ccatgggcgcgggccacggg

SEQ ID NO: 19458 - RNA, 20 nt, synthetic construct
  source 1..20: mol_type = other RNA
catgggcgcgggccacgggc

SEQ ID NO: 19459 - RNA, 20 nt, synthetic construct
  source 1..20: mol_type = other RNA
gggcgcgggccacgggcggg

SEQ ID NO: 19460 - RNA, 20 nt, synthetic construct
  source 1..20: mol_type = other RNA
ccgcccgtggcccgcgccca

SEQ ID NO: 19461 - RNA, 20 nt, synthetic construct
  source 1..20: mol_type = other RNA
gcgggccacgggcgggtggg

SEQ ID NO: 19462 - RNA, 20 nt, synthetic construct
  source 1..20: mol_type = other RNA
cgggccacgggcgggtggga

SEQ ID NO: 19463 - RNA, 20 nt, synthetic construct
  source 1..20: mol_type = other RNA
gccacgggcgggtgggaggg

SEQ ID NO: 19464 - RNA, 20 nt, synthetic construct
  source 1..20: mol_type = other RNA
ccacgggcgggtgggagggt

SEQ ID NO: 19465 - RNA, 20 nt, synthetic construct
  source 1..20: mol_type = other RNA
cacgggcgggtgggagggtg

SEQ ID NO: 19466 - RNA, 20 nt, synthetic construct
  source 1..20: mol_type = other RNA
acgggcgggtgggagggtgg

SEQ ID NO: 19467 - RNA, 20 nt, synthetic construct
  source 1..20: mol_type = other RNA
cgggcgggtgggagggtggg

SEQ ID NO: 19468 - RNA, 20 nt, synthetic construct
  source 1..20: mol_type = other RNA
cccaccctcccacccgcccg

SEQ ID NO: 19469 - RNA, 20 nt, synthetic construct
  source 1..20: mol_type = other RNA
gtgggagggtggggggccag

SEQ ID NO: 19470 - RNA, 20 nt, synthetic construct
  source 1..20: mol_type = other RNA
tgggagggtggggggccaga

SEQ ID NO: 19471 - RNA, 20 nt, synthetic construct
  source 1..20: mol_type = other RNA
gggagggtggggggccagag

SEQ ID NO: 19472 - RNA, 20 nt, synthetic construct
  source 1..20: mol_type = other RNA
agggtggggggccagagggg

SEQ ID NO: 19473 - RNA, 20 nt, synthetic construct
  source 1..20: mol_type = other RNA
gggtggggggccagaggggc

SEQ ID NO: 19474 - RNA, 20 nt, synthetic construct
  source 1..20: mol_type = other RNA
ggtggggggccagaggggcg

SEQ ID NO: 19475 - RNA, 20 nt, synthetic construct
  source 1..20: mol_type = other RNA
gtggggggccagaggggcgg

SEQ ID NO: 19476 - RNA, 20 nt, synthetic construct
  source 1..20: mol_type = other RNA
gggggccagaggggcggggg

SEQ ID NO: 19477 - RNA, 20 nt, synthetic construct
  source 1..20: mol_type = other RNA
ggggccagaggggcggggga

SEQ ID NO: 19478 - RNA, 20 nt, synthetic construct
  source 1..20: mol_type = other RNA
aggggcgggggagggtcact

SEQ ID NO: 19479 - RNA, 20 nt, synthetic construct
  source 1..20: mol_type = other RNA
gtgaccctcccccgcccctc

SEQ ID NO: 19480 - RNA, 20 nt, synthetic construct
  source 1..20: mol_type = other RNA
ggcgggggagggtcactcgg

SEQ ID NO: 19481 - RNA, 20 nt, synthetic construct
  source 1..20: mol_type = other RNA
gagggtcactcggcggctcc

SEQ ID NO: 19482 - RNA, 20 nt, synthetic construct
  source 1..20: mol_type = other RNA
tggcgggcggcggcggcacc

SEQ ID NO: 19483 - RNA, 20 nt, synthetic construct
  source 1..20: mol_type = other RNA
gtggcgggcggcggcggcac

SEQ ID NO: 19484 - RNA, 20 nt, synthetic construct
  source 1..20: mol_type = other RNA
gaggcggtggcgggcggcgg

SEQ ID NO: 19485 - RNA, 20 nt, synthetic construct
  source 1..20: mol_type = other RNA
gcagaggcggtggcgggcgg

SEQ ID NO: 19486 - RNA, 20 nt, synthetic construct
  source 1..20: mol_type = other RNA
ggagcagaggcggtggcggg

SEQ ID NO: 19487 - RNA, 20 nt, synthetic construct
  source 1..20: mol_type = other RNA
cggggagcagaggcggtggc

SEQ ID NO: 19488 - RNA, 20 nt, synthetic construct
  source 1..20: mol_type = other RNA
gcggggagcagaggcggtgg

SEQ ID NO: 19489 - RNA, 20 nt, synthetic construct
  source 1..20: mol_type = other RNA
cgcgcggggagcagaggcgg

SEQ ID NO: 19490 - RNA, 20 nt, synthetic construct
  source 1..20: mol_type = other RNA
gggcgcgcggggagcagagg

SEQ ID NO: 19491 - RNA, 20 nt, synthetic construct
  source 1..20: mol_type = other RNA
tgcgggcgcgcggggagcag

SEQ ID NO: 19492 - RNA, 20 nt, synthetic construct
  source 1..20: mol_type = other RNA
aacgtgtctgcgggcgcgcg

SEQ ID NO: 19493 - RNA, 20 nt, synthetic construct
  source 1..20: mol_type = other RNA
gaacgtgtctgcgggcgcgc

SEQ ID NO: 19494 - RNA, 20 nt, synthetic construct
  source 1..20: mol_type = other RNA
cgaacgtgtctgcgggcgcg

SEQ ID NO: 19495 - RNA, 20 nt, synthetic construct
  source 1..20: mol_type = other RNA
gcagacacgttcgttctctc

SEQ ID NO: 19496 - RNA, 20 nt, synthetic construct
  source 1..20: mol_type = other RNA
gagagaacgaacgtgtctgc

SEQ ID NO: 19497 - RNA, 20 nt, synthetic construct
  source 1..20: mol_type = other RNA
agagagaacgaacgtgtctg

SEQ ID NO: 19498 - RNA, 20 nt, synthetic construct
  source 1..20: mol_type = other RNA
acacgttcgttctctctggt

SEQ ID NO: 19499 - RNA, 20 nt, synthetic construct
  source 1..20: mol_type = other RNA
cacgttcgttctctctggtc

SEQ ID NO: 19500 - RNA, 20 nt, synthetic construct
  source 1..20: mol_type = other RNA
ctctctggtcgggaaactgc

SEQ ID NO: 19501 - RNA, 20 nt, synthetic construct
  source 1..20: mol_type = other RNA
gtcgggaaactgccggccgc

SEQ ID NO: 19502 - RNA, 20 nt, synthetic construct
  source 1..20: mol_type = other RNA
aaggaacgcgcgccggcggc

SEQ ID NO: 19503 - RNA, 20 nt, synthetic construct
  source 1..20: mol_type = other RNA
aagtaaggaacgcgcgccgg

SEQ ID NO: 19504 - RNA, 20 nt, synthetic construct
  source 1..20: mol_type = other RNA
tataagtaaggaacgcgcgc

SEQ ID NO: 19505 - RNA, 20 nt, synthetic construct
  source 1..20: mol_type = other RNA
agcgaaggaagttataagta

SEQ ID NO: 19506 - RNA, 20 nt, synthetic construct
  source 1..20: mol_type = other RNA
ggaggaaaaggctgtagcga

SEQ ID NO: 19507 - RNA, 20 nt, synthetic construct
  source 1..20: mol_type = other RNA
atgggagaaggcggaggaaa

SEQ ID NO: 19508 - RNA, 20 nt, synthetic construct
  source 1..20: mol_type = other RNA
cggggcatgggagaaggcgg

SEQ ID NO: 19509 - RNA, 20 nt, synthetic construct
  source 1..20: mol_type = other RNA
gggcggggcatgggagaagg

SEQ ID NO: 19510 - RNA, 20 nt, synthetic construct
  source 1..20: mol_type = other RNA
gaggggcggggcatgggaga

SEQ ID NO: 19511 - RNA, 20 nt, synthetic construct
  source 1..20: mol_type = other RNA
gaaagggaggggcggggcat

SEQ ID NO: 19512 - RNA, 20 nt, synthetic construct
  source 1..20: mol_type = other RNA
agaaagggaggggcggggca

SEQ ID NO: 19513 - RNA, 20 nt, synthetic construct
  source 1..20: mol_type = other RNA
agagaagaaagggaggggcg

SEQ ID NO: 19514 - RNA, 20 nt, synthetic construct
  source 1..20: mol_type = other RNA
gagagaagaaagggaggggc

SEQ ID NO: 19515 - RNA, 20 nt, synthetic construct
  source 1..20: mol_type = other RNA
ggagagaagaaagggagggg

SEQ ID NO: 19516 - RNA, 20 nt, synthetic construct
  source 1..20: mol_type = other RNA
ggcggagagaagaaagggag

SEQ ID NO: 19517 - RNA, 20 nt, synthetic construct
  source 1..20: mol_type = other RNA
gggcggagagaagaaaggga

SEQ ID NO: 19518 - RNA, 20 nt, synthetic construct
  source 1..20: mol_type = other RNA
ggggcggagagaagaaaggg

SEQ ID NO: 19519 - RNA, 20 nt, synthetic construct
  source 1..20: mol_type = other RNA
gggggggcggagagaagaaa

SEQ ID NO: 19520 - RNA, 20 nt, synthetic construct
  source 1..20: mol_type = other RNA
ggggggggcggagagaagaa

SEQ ID NO: 19521 - RNA, 20 nt, synthetic construct
  source 1..20: mol_type = other RNA
gaagggagcctcgggggggg

SEQ ID NO: 19522 - RNA, 20 nt, synthetic construct
  source 1..20: mol_type = other RNA
atggaagggagcctcggggg

SEQ ID NO: 19523 - RNA, 20 nt, synthetic construct
  source 1..20: mol_type = other RNA
gatggaagggagcctcgggg

SEQ ID NO: 19524 - RNA, 20 nt, synthetic construct
  source 1..20: mol_type = other RNA
cgatggaagggagcctcggg

SEQ ID NO: 19525 - RNA, 20 nt, synthetic construct
  source 1..20: mol_type = other RNA
acgatggaagggagcctcgg

SEQ ID NO: 19526 - RNA, 20 nt, synthetic construct
  source 1..20: mol_type = other RNA
aacgatggaagggagcctcg

SEQ ID NO: 19527 - RNA, 20 nt, synthetic construct
  source 1..20: mol_type = other RNA
caacgatggaagggagcctc

SEQ ID NO: 19528 - RNA, 20 nt, synthetic construct
  source 1..20: mol_type = other RNA
gctcccttccatcgttgcta

SEQ ID NO: 19529 - RNA, 20 nt, synthetic construct
  source 1..20: mol_type = other RNA
ctgccatagcaacgatggaa

SEQ ID NO: 19530 - RNA, 20 nt, synthetic construct
  source 1..20: mol_type = other RNA
gctgccatagcaacgatgga

SEQ ID NO: 19531 - RNA, 20 nt, synthetic construct
  source 1..20: mol_type = other RNA
tttagctgccatagcaacga

SEQ ID NO: 19532 - RNA, 20 nt, synthetic construct
  source 1..20: mol_type = other RNA
ggcagctaaatcaacaaact

SEQ ID NO: 19533 - RNA, 20 nt, synthetic construct
  source 1..20: mol_type = other RNA
atcaacaaactcggcgcacg

SEQ ID NO: 19534 - RNA, 20 nt, synthetic construct
  source 1..20: mol_type = other RNA
tcaacaaactcggcgcacgt

SEQ ID NO: 19535 - RNA, 20 nt, synthetic construct
  source 1..20: mol_type = other RNA
caacaaactcggcgcacgtg

SEQ ID NO: 19536 - RNA, 20 nt, synthetic construct
  source 1..20: mol_type = other RNA
aacaaactcggcgcacgtgg

SEQ ID NO: 19537 - RNA, 20 nt, synthetic construct
  source 1..20: mol_type = other RNA
aaactcggcgcacgtggggg

SEQ ID NO: 19538 - RNA, 20 nt, synthetic construct
  source 1..20: mol_type = other RNA
aactcggcgcacgtgggggc

SEQ ID NO: 19539 - RNA, 20 nt, synthetic construct
  source 1..20: mol_type = other RNA
actcggcgcacgtgggggcg

SEQ ID NO: 19540 - RNA, 20 nt, synthetic construct
  source 1..20: mol_type = other RNA
ctcggcgcacgtgggggcgg

SEQ ID NO: 19541 - RNA, 20 nt, synthetic construct
  source 1..20: mol_type = other RNA
ggcgcacgtgggggcggggg

SEQ ID NO: 19542 - RNA, 20 nt, synthetic construct
  source 1..20: mol_type = other RNA
gcgcacgtgggggcggggga

SEQ ID NO: 19543 - RNA, 20 nt, synthetic construct
  source 1..20: mol_type = other RNA
cgcacgtgggggcgggggag

SEQ ID NO: 19544 - RNA, 20 nt, synthetic construct
  source 1..20: mol_type = other RNA
cgtgggggcgggggagggga

SEQ ID NO: 19545 - RNA, 20 nt, synthetic construct
  source 1..20: mol_type = other RNA
gggggcgggggaggggaagg

SEQ ID NO: 19546 - RNA, 20 nt, synthetic construct
  source 1..20: mol_type = other RNA
ggggcgggggaggggaagga

SEQ ID NO: 19547 - RNA, 20 nt, synthetic construct
  source 1..20: mol_type = other RNA
gggcgggggaggggaaggag

SEQ ID NO: 19548 - RNA, 20 nt, synthetic construct
  source 1..20: mol_type = other RNA
ggggaggggaaggaggggcg

SEQ ID NO: 19549 - RNA, 20 nt, synthetic construct
  source 1..20: mol_type = other RNA
gggaggggaaggaggggcgc

SEQ ID NO: 19550 - RNA, 20 nt, synthetic construct
  source 1..20: mol_type = other RNA
aggggaaggaggggcgcggg

SEQ ID NO: 19551 - RNA, 20 nt, synthetic construct
  source 1..20: mol_type = other RNA
ggggaaggaggggcgcgggc

SEQ ID NO: 19552 - RNA, 20 nt, synthetic construct
  source 1..20: mol_type = other RNA
gggaaggaggggcgcgggcg

SEQ ID NO: 19553 - RNA, 20 nt, synthetic construct
  source 1..20: mol_type = other RNA
aggaggggcgcgggcggggc

SEQ ID NO: 19554 - RNA, 20 nt, synthetic construct
  source 1..20: mol_type = other RNA
ggaggggcgcgggcggggct

SEQ ID NO: 19555 - RNA, 20 nt, synthetic construct
  source 1..20: mol_type = other RNA
gggcgcgggcggggctgggc

SEQ ID NO: 19556 - RNA, 20 nt, synthetic construct
  source 1..20: mol_type = other RNA
ggcgcgggcggggctgggcc

SEQ ID NO: 19557 - RNA, 20 nt, synthetic construct
  source 1..20: mol_type = other RNA
gccgggccgtgacgccagcc

SEQ ID NO: 19558 - RNA, 20 nt, synthetic construct
  source 1..20: mol_type = other RNA
gcctggctggcgtcacggcc

SEQ ID NO: 19559 - RNA, 20 nt, synthetic construct
  source 1..20: mol_type = other RNA
cgtgacgccagccaggcagc

SEQ ID NO: 19560 - RNA, 20 nt, synthetic construct
  source 1..20: mol_type = other RNA
gacgccagccaggcagctgg

SEQ ID NO: 19561 - RNA, 20 nt, synthetic construct
  source 1..20: mol_type = other RNA
cagctgcctggctggcgtca

SEQ ID NO: 19562 - RNA, 20 nt, synthetic construct
  source 1..20: mol_type = other RNA
cagccaggcagctggcgggc

SEQ ID NO: 19563 - RNA, 20 nt, synthetic construct
  source 1..20: mol_type = other RNA
cagcccgccagctgcctggc

SEQ ID NO: 19564 - RNA, 20 nt, synthetic construct
  source 1..20: mol_type = other RNA
gctccagcccgccagctgcc

SEQ ID NO: 19565 - RNA, 20 nt, synthetic construct
  source 1..20: mol_type = other RNA
ggctggagccgagctgacgc

SEQ ID NO: 19566 - RNA, 20 nt, synthetic construct
  source 1..20: mol_type = other RNA
tggagccgagctgacgccgg

SEQ ID NO: 19567 - RNA, 20 nt, synthetic construct
  source 1..20: mol_type = other RNA
cgagctgacgccggcggcag

SEQ ID NO: 19568 - RNA, 20 nt, synthetic construct
  source 1..20: mol_type = other RNA
cactgccgccggcgtcagct

SEQ ID NO: 19569 - RNA, 20 nt, synthetic construct
  source 1..20: mol_type = other RNA
gacgccggcggcagtggtgt

SEQ ID NO: 19570 - RNA, 20 nt, synthetic construct
  source 1..20: mol_type = other RNA
gccggcggcagtggtgtcgg

SEQ ID NO: 19571 - RNA, 20 nt, synthetic construct
  source 1..20: mol_type = other RNA
ggcggcagtggtgtcggcgg

SEQ ID NO: 19572 - RNA, 20 nt, synthetic construct
  source 1..20: mol_type = other RNA
gccgccgacaccactgccgc

SEQ ID NO: 19573 - RNA, 20 nt, synthetic construct
  source 1..20: mol_type = other RNA
agtggtgtcggcggcggcgg

SEQ ID NO: 19574 - RNA, 20 nt, synthetic construct
  source 1..20: mol_type = other RNA
cggcggcgtccgccccagcg

SEQ ID NO: 19575 - RNA, 20 nt, synthetic construct
  source 1..20: mol_type = other RNA
ggcggcgtccgccccagcgc

SEQ ID NO: 19576 - RNA, 20 nt, synthetic construct
  source 1..20: mol_type = other RNA
gcggcgtccgccccagcgcg

SEQ ID NO: 19577 - RNA, 20 nt, synthetic construct
  source 1..20: mol_type = other RNA
ccgccccagcgcggggcgcg

SEQ ID NO: 19578 - RNA, 20 nt, synthetic construct
  source 1..20: mol_type = other RNA
cctcgcgccccgcgctgggg

SEQ ID NO: 19579 - RNA, 20 nt, synthetic construct
  source 1..20: mol_type = other RNA
cagcgcggggcgcgaggaac

SEQ ID NO: 19580 - RNA, 20 nt, synthetic construct
  source 1..20: mol_type = other RNA
agcgcggggcgcgaggaacc

SEQ ID NO: 19581 - RNA, 20 nt, synthetic construct
  source 1..20: mol_type = other RNA
gttcctcgcgccccgcgctg

SEQ ID NO: 19582 - RNA, 20 nt, synthetic construct
  source 1..20: mol_type = other RNA
ggttcctcgcgccccgcgct

SEQ ID NO: 19583 - RNA, 20 nt, synthetic construct
  source 1..20: mol_type = other RNA
cggttcctcgcgccccgcgc

SEQ ID NO: 19584 - RNA, 20 nt, synthetic construct
  source 1..20: mol_type = other RNA
gggcgcgaggaaccgggcgc

SEQ ID NO: 19585 - RNA, 20 nt, synthetic construct
  source 1..20: mol_type = other RNA
cgaggaaccgggcgcaggtt

SEQ ID NO: 19586 - RNA, 20 nt, synthetic construct
  source 1..20: mol_type = other RNA
gcagcgaccgaacctgcgcc

SEQ ID NO: 19587 - RNA, 20 nt, synthetic construct
  source 1..20: mol_type = other RNA
ggttcggtcgctgcgcgacc

SEQ ID NO: 19588 - RNA, 20 nt, synthetic construct
  source 1..20: mol_type = other RNA
gttcggtcgctgcgcgacca

SEQ ID NO: 19589 - RNA, 20 nt, synthetic construct
  source 1..20: mol_type = other RNA
gccgtactcaccgccattgt

SEQ ID NO: 19590 - RNA, 20 nt, synthetic construct
  source 1..20: mol_type = other RNA
gccgacaatggcggtgagta

SEQ ID NO: 19591 - RNA, 20 nt, synthetic construct
  source 1..20: mol_type = other RNA
caccgccattgtcggctccc

SEQ ID NO: 19592 - RNA, 20 nt, synthetic construct
  source 1..20: mol_type = other RNA
accgccattgtcggctccct

SEQ ID NO: 19593 - RNA, 20 nt, synthetic construct
  source 1..20: mol_type = other RNA
acccagggagccgacaatgg

SEQ ID NO: 19594 - RNA, 20 nt, synthetic construct
  source 1..20: mol_type = other RNA
cgaacccagggagccgacaa

SEQ ID NO: 19595 - RNA, 20 nt, synthetic construct
  source 1..20: mol_type = other RNA
cttcgcgggcttcgaaccca

SEQ ID NO: 19596 - RNA, 20 nt, synthetic construct
  source 1..20: mol_type = other RNA
tcttcgcgggcttcgaaccc

SEQ ID NO: 19597 - RNA, 20 nt, synthetic construct
  source 1..20: mol_type = other RNA
tcgaagcccgcgaagactgg

SEQ ID NO: 19598 - RNA, 20 nt, synthetic construct
  source 1..20: mol_type = other RNA
cgaagcccgcgaagactggt

SEQ ID NO: 19599 - RNA, 20 nt, synthetic construct
  source 1..20: mol_type = other RNA
gaagcccgcgaagactggtg

SEQ ID NO: 19600 - RNA, 20 nt, synthetic construct
  source 1..20: mol_type = other RNA
gcgaagactggtggggtcag

SEQ ID NO: 19601 - RNA, 20 nt, synthetic construct
  source 1..20: mol_type = other RNA
cgaagactggtggggtcagc

SEQ ID NO: 19602 - RNA, 20 nt, synthetic construct
  source 1..20: mol_type = other RNA
ctgaccccaccagtcttcgc

SEQ ID NO: 19603 - RNA, 20 nt, synthetic construct
  source 1..20: mol_type = other RNA
gctgaccccaccagtcttcg

SEQ ID NO: 19604 - RNA, 20 nt, synthetic construct
  source 1..20: mol_type = other RNA
agactggtggggtcagcggg

SEQ ID NO: 19605 - RNA, 20 nt, synthetic construct
  source 1..20: mol_type = other RNA
ggtggggtcagcgggcggca

SEQ ID NO: 19606 - RNA, 20 nt, synthetic construct
  source 1..20: mol_type = other RNA
cgcgtatgctagcaggggtg

SEQ ID NO: 19607 - RNA, 20 nt, synthetic construct
  source 1..20: mol_type = other RNA
gcaagcgcgtatgctagcag

SEQ ID NO: 19608 - RNA, 20 nt, synthetic construct
  source 1..20: mol_type = other RNA
ggcaagcgcgtatgctagca

SEQ ID NO: 19609 - RNA, 20 nt, synthetic construct
  source 1..20: mol_type = other RNA
cggcaagcgcgtatgctagc

SEQ ID NO: 19610 - RNA, 20 nt, synthetic construct
  source 1..20: mol_type = other RNA
ttgccgcgctgtctgcgcgc

SEQ ID NO: 19611 - RNA, 20 nt, synthetic construct
  source 1..20: mol_type = other RNA
tctccagcgcgcagacagcg

SEQ ID NO: 19612 - RNA, 20 nt, synthetic construct
  source 1..20: mol_type = other RNA
ggagggctggatgagtcacg

SEQ ID NO: 19613 - RNA, 20 nt, synthetic construct
  source 1..20: mol_type = other RNA
gggagggggagatggagggc

SEQ ID NO: 19614 - RNA, 20 nt, synthetic construct
  source 1..20: mol_type = other RNA
gagagggagggggagatgga

SEQ ID NO: 19615 - RNA, 20 nt, synthetic construct
  source 1..20: mol_type = other RNA
agagagggagggggagatgg

SEQ ID NO: 19616 - RNA, 20 nt, synthetic construct
  source 1..20: mol_type = other RNA
cgcagagagggagggggaga

SEQ ID NO: 19617 - RNA, 20 nt, synthetic construct
  source 1..20: mol_type = other RNA
ccctccctctctgcgctcgc

SEQ ID NO: 19618 - RNA, 20 nt, synthetic construct
  source 1..20: mol_type = other RNA
tgcgagcgcagagagggagg

SEQ ID NO: 19619 - RNA, 20 nt, synthetic construct
  source 1..20: mol_type = other RNA
ctgcgagcgcagagagggag

SEQ ID NO: 19620 - RNA, 20 nt, synthetic construct
  source 1..20: mol_type = other RNA
cctgcgagcgcagagaggga

SEQ ID NO: 19621 - RNA, 20 nt, synthetic construct
  source 1..20: mol_type = other RNA
tcctgcgagcgcagagaggg

SEQ ID NO: 19622 - RNA, 20 nt, synthetic construct
  source 1..20: mol_type = other RNA
gactcctgcgagcgcagaga

SEQ ID NO: 19623 - RNA, 20 nt, synthetic construct
  source 1..20: mol_type = other RNA
ggactcctgcgagcgcagag

SEQ ID NO: 19624 - RNA, 20 nt, synthetic construct
  source 1..20: mol_type = other RNA
ctggcgctgagcgacgagag

SEQ ID NO: 19625 - RNA, 20 nt, synthetic construct
  source 1..20: mol_type = other RNA
tcgtcgctcagcgccagtgc

SEQ ID NO: 19626 - RNA, 20 nt, synthetic construct
  source 1..20: mol_type = other RNA
tcgctcagcgccagtgccgg

SEQ ID NO: 19627 - RNA, 20 nt, synthetic construct
  source 1..20: mol_type = other RNA
ctcagcgccagtgccggtgg

SEQ ID NO: 19628 - RNA, 20 nt, synthetic construct
  source 1..20: mol_type = other RNA
gccagtgccggtggcggtgc

SEQ ID NO: 19629 - RNA, 20 nt, synthetic construct
  source 1..20: mol_type = other RNA
gccggcaccgccaccggcac

SEQ ID NO: 19630 - RNA, 20 nt, synthetic construct
  source 1..20: mol_type = other RNA
ccggtggcggtgccggcgct

SEQ ID NO: 19631 - RNA, 20 nt, synthetic construct
  source 1..20: mol_type = other RNA
ccgagcgccggcaccgccac

SEQ ID NO: 19632 - RNA, 20 nt, synthetic construct
  source 1..20: mol_type = other RNA
gcgctcggcctgacctcgca

SEQ ID NO: 19633 - RNA, 20 nt, synthetic construct
  source 1..20: mol_type = other RNA
tgcgaggtcaggccgagcgc

SEQ ID NO: 19634 - RNA, 20 nt, synthetic construct
  source 1..20: mol_type = other RNA
tgacctcgcacggttcctcg

SEQ ID NO: 19635 - RNA, 20 nt, synthetic construct
  source 1..20: mol_type = other RNA
gacctcgcacggttcctcgc

SEQ ID NO: 19636 - RNA, 20 nt, synthetic construct
  source 1..20: mol_type = other RNA
gcgaggaaccgtgcgaggtc

SEQ ID NO: 19637 - RNA, 20 nt, synthetic construct
  source 1..20: mol_type = other RNA
ggcccgcgaggaaccgtgcg

SEQ ID NO: 19638 - RNA, 20 nt, synthetic construct
  source 1..20: mol_type = other RNA
cctcgcgggcccttctgctg

SEQ ID NO: 19639 - RNA, 20 nt, synthetic construct
  source 1..20: mol_type = other RNA
ctcgcgggcccttctgctga

SEQ ID NO: 19640 - RNA, 20 nt, synthetic construct
  source 1..20: mol_type = other RNA
tcgcgggcccttctgctgag

SEQ ID NO: 19641 - RNA, 20 nt, synthetic construct
  source 1..20: mol_type = other RNA
cgggcccttctgctgagggg

SEQ ID NO: 19642 - RNA, 20 nt, synthetic construct
  source 1..20: mol_type = other RNA
gggcccttctgctgaggggt

SEQ ID NO: 19643 - RNA, 20 nt, synthetic construct
  source 1..20: mol_type = other RNA
ggcccttctgctgaggggtg

SEQ ID NO: 19644 - RNA, 20 nt, synthetic construct
  source 1..20: mol_type = other RNA
gcccttctgctgaggggtgg

SEQ ID NO: 19645 - RNA, 20 nt, synthetic construct
  source 1..20: mol_type = other RNA
cccttctgctgaggggtggg

SEQ ID NO: 19646 - RNA, 20 nt, synthetic construct
  source 1..20: mol_type = other RNA
ccccccacccctcagcagaa

SEQ ID NO: 19647 - RNA, 20 nt, synthetic construct
  source 1..20: mol_type = other RNA
gccccccacccctcagcaga

SEQ ID NO: 19648 - RNA, 20 nt, synthetic construct
  source 1..20: mol_type = other RNA
gctgaggggtggggggcgct

SEQ ID NO: 19649 - RNA, 20 nt, synthetic construct
  source 1..20: mol_type = other RNA
ctgaggggtggggggcgcta

SEQ ID NO: 19650 - RNA, 20 nt, synthetic construct
  source 1..20: mol_type = other RNA
tgaggggtggggggcgctag

SEQ ID NO: 19651 - RNA, 20 nt, synthetic construct
  source 1..20: mol_type = other RNA
ggtggggggcgctaggggtg

SEQ ID NO: 19652 - RNA, 20 nt, synthetic construct
  source 1..20: mol_type = other RNA
ggggcgctaggggtgtggag

SEQ ID NO: 19653 - RNA, 20 nt, synthetic construct
  source 1..20: mol_type = other RNA
gcgctaggggtgtggagagg

SEQ ID NO: 19654 - RNA, 20 nt, synthetic construct
  source 1..20: mol_type = other RNA
cagcactgtgcagcgtgaac

SEQ ID NO: 19655 - RNA, 20 nt, synthetic construct
  source 1..20: mol_type = other RNA
agcactgtgcagcgtgaact

SEQ ID NO: 19656 - RNA, 20 nt, synthetic construct
  source 1..20: mol_type = other RNA
agttcacgctgcacagtgct

SEQ ID NO: 19657 - RNA, 20 nt, synthetic construct
  source 1..20: mol_type = other RNA
cagttcacgctgcacagtgc

SEQ ID NO: 19658 - RNA, 20 nt, synthetic construct
  source 1..20: mol_type = other RNA
gaactgggagcctcaagaga

SEQ ID NO: 19659 - RNA, 20 nt, synthetic construct
  source 1..20: mol_type = other RNA
gagcctcaagagaaggccag

SEQ ID NO: 19660 - RNA, 20 nt, synthetic construct
  source 1..20: mol_type = other RNA
actcctctggccttctcttg

SEQ ID NO: 19661 - RNA, 20 nt, synthetic construct
  source 1..20: mol_type = other RNA
aggccagaggagtgttccgc

SEQ ID NO: 19662 - RNA, 20 nt, synthetic construct
  source 1..20: mol_type = other RNA
ggccagaggagtgttccgcc

SEQ ID NO: 19663 - RNA, 20 nt, synthetic construct
  source 1..20: mol_type = other RNA
aggagtgttccgccgggaac

SEQ ID NO: 19664 - RNA, 20 nt, synthetic construct
  source 1..20: mol_type = other RNA
ttcccggcggaacactcctc

SEQ ID NO: 19665 - RNA, 20 nt, synthetic construct
  source 1..20: mol_type = other RNA
agtgttccgccgggaacagg

SEQ ID NO: 19666 - RNA, 20 nt, synthetic construct
  source 1..20: mol_type = other RNA
cgccgggaacaggcggaaag

SEQ ID NO: 19667 - RNA, 20 nt, synthetic construct
  source 1..20: mol_type = other RNA
ctctttccgcctgttcccgg

SEQ ID NO: 19668 - RNA, 20 nt, synthetic construct
  source 1..20: mol_type = other RNA
tgcctctttccgcctgttcc

SEQ ID NO: 19669 - RNA, 20 nt, synthetic construct
  source 1..20: mol_type = other RNA
caggcggaaagaggcacgaa

SEQ ID NO: 19670 - RNA, 20 nt, synthetic construct
  source 1..20: mol_type = other RNA
aggcggaaagaggcacgaat

SEQ ID NO: 19671 - RNA, 20 nt, synthetic construct
  source 1..20: mol_type = other RNA
ggcggaaagaggcacgaatg

SEQ ID NO: 19672 - RNA, 20 nt, synthetic construct
  source 1..20: mol_type = other RNA
gaggcacgaatggggagtta

SEQ ID NO: 19673 - RNA, 20 nt, synthetic construct
  source 1..20: mol_type = other RNA
gatactttaaatagcgagaa

SEQ ID NO: 19674 - RNA, 20 nt, synthetic construct
  source 1..20: mol_type = other RNA
atactttaaatagcgagaaa

SEQ ID NO: 19675 - RNA, 20 nt, synthetic construct
  source 1..20: mol_type = other RNA
atagcgagaaagggagtgaa

SEQ ID NO: 19676 - RNA, 20 nt, synthetic construct
  source 1..20: mol_type = other RNA
tagcgagaaagggagtgaaa

SEQ ID NO: 19677 - RNA, 20 nt, synthetic construct
  source 1..20: mol_type = other RNA
agggctcaagatttactcag

SEQ ID NO: 19678 - RNA, 20 nt, synthetic construct
  source 1..20: mol_type = other RNA
aagatttactcagaggcata

SEQ ID NO: 19679 - RNA, 20 nt, synthetic construct
  source 1..20: mol_type = other RNA
agatttactcagaggcataa

SEQ ID NO: 19680 - RNA, 20 nt, synthetic construct
  source 1..20: mol_type = other RNA
agaggcataagggagagaag

SEQ ID NO: 19681 - RNA, 20 nt, synthetic construct
  source 1..20: mol_type = other RNA
gaggcataagggagagaaga

SEQ ID NO: 19682 - RNA, 20 nt, synthetic construct
  source 1..20: mol_type = other RNA
gggagagaagagggactgtg

SEQ ID NO: 19683 - RNA, 20 nt, synthetic construct
  source 1..20: mol_type = other RNA
agaagagggactgtgaggcg

SEQ ID NO: 19684 - RNA, 20 nt, synthetic construct
  source 1..20: mol_type = other RNA
ggaaagggcttcgagatggc

SEQ ID NO: 19685 - RNA, 20 nt, synthetic construct
  source 1..20: mol_type = other RNA
aaaaggaaagggcttcgaga

SEQ ID NO: 19686 - RNA, 20 nt, synthetic construct
  source 1..20: mol_type = other RNA
agaaagaaaaaaaaaggaaa

SEQ ID NO: 19687 - RNA, 20 nt, synthetic construct
  source 1..20: mol_type = other RNA
aagaaagaaaaaaaaaggaa

SEQ ID NO: 19688 - RNA, 20 nt, synthetic construct
  source 1..20: mol_type = other RNA
aaaaaaagaaagaaaaaaaa

SEQ ID NO: 19689 - RNA, 20 nt, synthetic construct
  source 1..20: mol_type = other RNA
tctcgctgtgtcgcccaagc

SEQ ID NO: 19690 - RNA, 20 nt, synthetic construct
  source 1..20: mol_type = other RNA
tcgcccaagctggaatgcag

SEQ ID NO: 19691 - RNA, 20 nt, synthetic construct
  source 1..20: mol_type = other RNA
gtgccactgcattccagctt

SEQ ID NO: 19692 - RNA, 20 nt, synthetic construct
  source 1..20: mol_type = other RNA
cgtgccactgcattccagct

SEQ ID NO: 19693 - RNA, 20 nt, synthetic construct
  source 1..20: mol_type = other RNA
cgcttggacgcaggaggcgg

SEQ ID NO: 19694 - RNA, 20 nt, synthetic construct
  source 1..20: mol_type = other RNA
aatcgcttggacgcaggagg

SEQ ID NO: 19695 - RNA, 20 nt, synthetic construct
  source 1..20: mol_type = other RNA
gagaatcgcttggacgcagg

SEQ ID NO: 19696 - RNA, 20 nt, synthetic construct
  source 1..20: mol_type = other RNA
caggagaatcgcttggacgc

SEQ ID NO: 19697 - RNA, 20 nt, synthetic construct
  source 1..20: mol_type = other RNA
gctgacgcaggagaatcgct

SEQ ID NO: 19698 - RNA, 20 nt, synthetic construct
  source 1..20: mol_type = other RNA
tgcgtcagcctcccgagtag

SEQ ID NO: 19699 - RNA, 20 nt, synthetic construct
  source 1..20: mol_type = other RNA
gcgtcagcctcccgagtagc

SEQ ID NO: 19700 - RNA, 20 nt, synthetic construct
  source 1..20: mol_type = other RNA
cgtcagcctcccgagtagcg

SEQ ID NO: 19701 - RNA, 20 nt, synthetic construct
  source 1..20: mol_type = other RNA
gctactcgggaggctgacgc

SEQ ID NO: 19702 - RNA, 20 nt, synthetic construct
  source 1..20: mol_type = other RNA
tcccgagtagcggggattac

SEQ ID NO: 19703 - RNA, 20 nt, synthetic construct
  source 1..20: mol_type = other RNA
tgtaatccccgctactcggg

SEQ ID NO: 19704 - RNA, 20 nt, synthetic construct
  source 1..20: mol_type = other RNA
gcctgtaatccccgctactc

SEQ ID NO: 19705 - RNA, 20 nt, synthetic construct
  source 1..20: mol_type = other RNA
cgcctgtaatccccgctact

SEQ ID NO: 19706 - RNA, 20 nt, synthetic construct
  source 1..20: mol_type = other RNA
acaggcgtgcgccacgacgc

SEQ ID NO: 19707 - RNA, 20 nt, synthetic construct
  source 1..20: mol_type = other RNA
acaaaaattagccggcgtcg

SEQ ID NO: 19708 - RNA, 20 nt, synthetic construct
  source 1..20: mol_type = other RNA
gctaatttttgtatttttcg

SEQ ID NO: 19709 - RNA, 20 nt, synthetic construct
  source 1..20: mol_type = other RNA
cgaaaaatacaaaaattagc

SEQ ID NO: 19710 - RNA, 20 nt, synthetic construct
  source 1..20: mol_type = other RNA
ttttgtatttttcgtggaga

SEQ ID NO: 19711 - RNA, 20 nt, synthetic construct
  source 1..20: mol_type = other RNA
tttgtatttttcgtggagac

SEQ ID NO: 19712 - RNA, 20 nt, synthetic construct
  source 1..20: mol_type = other RNA
ttgtatttttcgtggagacg

SEQ ID NO: 19713 - RNA, 20 nt, synthetic construct
  source 1..20: mol_type = other RNA
gagacggggtttcaccatgt

SEQ ID NO: 19714 - RNA, 20 nt, synthetic construct
  source 1..20: mol_type = other RNA
ggggtttcaccatgttggcc

SEQ ID NO: 19715 - RNA, 20 nt, synthetic construct
  source 1..20: mol_type = other RNA
tttcaccatgttggccaggc

SEQ ID NO: 19716 - RNA, 20 nt, synthetic construct
  source 1..20: mol_type = other RNA
cgagacctgcctggccaaca

SEQ ID NO: 19717 - RNA, 20 nt, synthetic construct
  source 1..20: mol_type = other RNA
tcaggtgttcgagacctgcc

SEQ ID NO: 19718 - RNA, 20 nt, synthetic construct
  source 1..20: mol_type = other RNA
caggctgatcacttgaggtc

SEQ ID NO: 19719 - RNA, 20 nt, synthetic construct
  source 1..20: mol_type = other RNA
ctcaagtgatcagcctgcct

SEQ ID NO: 19720 - RNA, 20 nt, synthetic construct
  source 1..20: mol_type = other RNA
cgaggcaggctgatcacttg

SEQ ID NO: 19721 - RNA, 20 nt, synthetic construct
  source 1..20: mol_type = other RNA
gcctcggcctcccgaagtgc

SEQ ID NO: 19722 - RNA, 20 nt, synthetic construct
  source 1..20: mol_type = other RNA
cctcggcctcccgaagtgct

SEQ ID NO: 19723 - RNA, 20 nt, synthetic construct
  source 1..20: mol_type = other RNA
gcacttcgggaggccgaggc

SEQ ID NO: 19724 - RNA, 20 nt, synthetic construct
  source 1..20: mol_type = other RNA
cccagcacttcgggaggccg

SEQ ID NO: 19725 - RNA, 20 nt, synthetic construct
  source 1..20: mol_type = other RNA
tcccgaagtgctgggattac

SEQ ID NO: 19726 - RNA, 20 nt, synthetic construct
  source 1..20: mol_type = other RNA
tgtaatcccagcacttcggg

SEQ ID NO: 19727 - RNA, 20 nt, synthetic construct
  source 1..20: mol_type = other RNA
gcctgtaatcccagcacttc

SEQ ID NO: 19728 - RNA, 20 nt, synthetic construct
  source 1..20: mol_type = other RNA
cgcctgtaatcccagcactt

SEQ ID NO: 19729 - RNA, 20 nt, synthetic construct
  source 1..20: mol_type = other RNA
tcatcaaatattacaggcag

SEQ ID NO: 19730 - RNA, 20 nt, synthetic construct
  source 1..20: mol_type = other RNA
atttagtcatcaaatattac

SEQ ID NO: 19731 - RNA, 20 nt, synthetic construct
  source 1..20: mol_type = other RNA
gtgtttaattcttctttaat

SEQ ID NO: 19732 - RNA, 20 nt, synthetic construct
  source 1..20: mol_type = other RNA
agtgtttaattcttctttaa

SEQ ID NO: 19733 - RNA, 20 nt, synthetic construct
  source 1..20: mol_type = other RNA
gcactctcctttccacttta

SEQ ID NO: 19734 - RNA, 20 nt, synthetic construct
  source 1..20: mol_type = other RNA
aaagtggaaaggagagtgcg

SEQ ID NO: 19735 - RNA, 20 nt, synthetic construct
  source 1..20: mol_type = other RNA
ttctcatccataaagtggaa

SEQ ID NO: 19736 - RNA, 20 nt, synthetic construct
  source 1..20: mol_type = other RNA
tcaatttctcatccataaag

SEQ ID NO: 19737 - RNA, 20 nt, synthetic construct
  source 1..20: mol_type = other RNA
tgagaaattgagtcataaag

SEQ ID NO: 19738 - RNA, 20 nt, synthetic construct
  source 1..20: mol_type = other RNA
tgagtcataaagaggtgaaa

SEQ ID NO: 19739 - RNA, 20 nt, synthetic construct
  source 1..20: mol_type = other RNA
agaggtgaaatggccagtaa

SEQ ID NO: 19740 - RNA, 20 nt, synthetic construct
  source 1..20: mol_type = other RNA
aaatggccagtaaaggtcaa

SEQ ID NO: 19741 - RNA, 20 nt, synthetic construct
  source 1..20: mol_type = other RNA
agttgtcctttgacctttac

SEQ ID NO: 19742 - RNA, 20 nt, synthetic construct
  source 1..20: mol_type = other RNA
caaaggacaactcgttcctt

SEQ ID NO: 19743 - RNA, 20 nt, synthetic construct
  source 1..20: mol_type = other RNA
acaactcgttccttcggctc

SEQ ID NO: 19744 - RNA, 20 nt, synthetic construct
  source 1..20: mol_type = other RNA
cgttccttcggctcaggctc

SEQ ID NO: 19745 - RNA, 20 nt, synthetic construct
  source 1..20: mol_type = other RNA
gttccttcggctcaggctcc

SEQ ID NO: 19746 - RNA, 20 nt, synthetic construct
  source 1..20: mol_type = other RNA
cttcggctcaggctccgggt

SEQ ID NO: 19747 - RNA, 20 nt, synthetic construct
  source 1..20: mol_type = other RNA
ctacccggagcctgagccga

SEQ ID NO: 19748 - RNA, 20 nt, synthetic construct
  source 1..20: mol_type = other RNA
gctcaggctccgggtaggtc

SEQ ID NO: 19749 - RNA, 20 nt, synthetic construct
  source 1..20: mol_type = other RNA
ggtaggtcaggcccccctaa

SEQ ID NO: 19750 - RNA, 20 nt, synthetic construct
  source 1..20: mol_type = other RNA
gtaggtcaggcccccctaaa

SEQ ID NO: 19751 - RNA, 20 nt, synthetic construct
  source 1..20: mol_type = other RNA
ttaggggggcctgacctacc

SEQ ID NO: 19752 - RNA, 20 nt, synthetic construct
  source 1..20: mol_type = other RNA
cccccctaaagggacttccc

SEQ ID NO: 19753 - RNA, 20 nt, synthetic construct
  source 1..20: mol_type = other RNA
ccccctaaagggacttccct

SEQ ID NO: 19754 - RNA, 20 nt, synthetic construct
  source 1..20: mol_type = other RNA
ccagggaagtccctttaggg

SEQ ID NO: 19755 - RNA, 20 nt, synthetic construct
  source 1..20: mol_type = other RNA
cccagggaagtccctttagg

SEQ ID NO: 19756 - RNA, 20 nt, synthetic construct
  source 1..20: mol_type = other RNA
tcccagggaagtccctttag

SEQ ID NO: 19757 - RNA, 20 nt, synthetic construct
  source 1..20: mol_type = other RNA
ttcccagggaagtcccttta

SEQ ID NO: 19758 - RNA, 20 nt, synthetic construct
  source 1..20: mol_type = other RNA
cttcccagggaagtcccttt

SEQ ID NO: 19759 - RNA, 20 nt, synthetic construct
  source 1..20: mol_type = other RNA
ctgggaagtgaccatgtgcc

SEQ ID NO: 19760 - RNA, 20 nt, synthetic construct
  source 1..20: mol_type = other RNA
tggcacatggtcacttccca

SEQ ID NO: 19761 - RNA, 20 nt, synthetic construct
  source 1..20: mol_type = other RNA
ctggcacatggtcacttccc

SEQ ID NO: 19762 - RNA, 20 nt, synthetic construct
  source 1..20: mol_type = other RNA
agtgaccatgtgccaggaag

SEQ ID NO: 19763 - RNA, 20 nt, synthetic construct
  source 1..20: mol_type = other RNA
tcgctccacttcctggcaca

SEQ ID NO: 19764 - RNA, 20 nt, synthetic construct
  source 1..20: mol_type = other RNA
caggaagtggagcgatgcgg

SEQ ID NO: 19765 - RNA, 20 nt, synthetic construct
  source 1..20: mol_type = other RNA
aggaagtggagcgatgcggt

SEQ ID NO: 19766 - RNA, 20 nt, synthetic construct
  source 1..20: mol_type = other RNA
caccgcatcgctccacttcc

SEQ ID NO: 19767 - RNA, 20 nt, synthetic construct
  source 1..20: mol_type = other RNA
gtgtgcactttttgagagct

SEQ ID NO: 19768 - RNA, 20 nt, synthetic construct
  source 1..20: mol_type = other RNA
gtgcacaccgagcccgccgc

SEQ ID NO: 19769 - RNA, 20 nt, synthetic construct
  source 1..20: mol_type = other RNA
aaggacgcctgcggcgggct

SEQ ID NO: 19770 - RNA, 20 nt, synthetic construct
  source 1..20: mol_type = other RNA
tgggcaaggacgcctgcggc

SEQ ID NO: 19771 - RNA, 20 nt, synthetic construct
  source 1..20: mol_type = other RNA
gtgggcaaggacgcctgcgg

SEQ ID NO: 19772 - RNA, 20 nt, synthetic construct
  source 1..20: mol_type = other RNA
ccggtgggcaaggacgcctg

SEQ ID NO: 19773 - RNA, 20 nt, synthetic construct
  source 1..20: mol_type = other RNA
cccagctactcgggaggctg

SEQ ID NO: 19774 - RNA, 20 nt, synthetic construct
  source 1..20: mol_type = other RNA
gctactcgggaggctgaggt

SEQ ID NO: 19775 - RNA, 20 nt, synthetic construct
  source 1..20: mol_type = other RNA
actcgggaggctgaggtagg

SEQ ID NO: 19776 - RNA, 20 nt, synthetic construct
  source 1..20: mol_type = other RNA
ctcgggaggctgaggtagga

SEQ ID NO: 19777 - RNA, 20 nt, synthetic construct
  source 1..20: mol_type = other RNA
taggagggttgcttaagccc

SEQ ID NO: 19778 - RNA, 20 nt, synthetic construct
  source 1..20: mol_type = other RNA
ccaggagttcaagaccagcc

SEQ ID NO: 19779 - RNA, 20 nt, synthetic construct
  source 1..20: mol_type = other RNA
caggctggtcttgaactcct

SEQ ID NO: 19780 - RNA, 20 nt, synthetic construct
  source 1..20: mol_type = other RNA
ccaggctggtcttgaactcc

SEQ ID NO: 19781 - RNA, 20 nt, synthetic construct
  source 1..20: mol_type = other RNA
tctcactatgttgtccaggc

SEQ ID NO: 19782 - RNA, 20 nt, synthetic construct
  source 1..20: mol_type = other RNA
agggtctcactatgttgtcc

SEQ ID NO: 19783 - RNA, 20 nt, synthetic construct
  source 1..20: mol_type = other RNA
tctttttgctgtttgagaca

SEQ ID NO: 19784 - RNA, 20 nt, synthetic construct
  source 1..20: mol_type = other RNA
ctctttttgctgtttgagac

SEQ ID NO: 19785 - RNA, 20 nt, synthetic construct
  source 1..20: mol_type = other RNA
caaaaagagtagatctcctt

SEQ ID NO: 19786 - RNA, 20 nt, synthetic construct
  source 1..20: mol_type = other RNA
tctcctttggttctaacaag

SEQ ID NO: 19787 - RNA, 20 nt, synthetic construct
  source 1..20: mol_type = other RNA
ctcctttggttctaacaaga

SEQ ID NO: 19788 - RNA, 20 nt, synthetic construct
  source 1..20: mol_type = other RNA
tcctttggttctaacaagag

SEQ ID NO: 19789 - RNA, 20 nt, synthetic construct
  source 1..20: mol_type = other RNA
tcccctcttgttagaaccaa

SEQ ID NO: 19790 - RNA, 20 nt, synthetic construct
  source 1..20: mol_type = other RNA
aagacagcagagtggacagt

SEQ ID NO: 19791 - RNA, 20 nt, synthetic construct
  source 1..20: mol_type = other RNA
aaagacagcagagtggacag

SEQ ID NO: 19792 - RNA, 20 nt, synthetic construct
  source 1..20: mol_type = other RNA
tctgctgtcttttcgtgcct

SEQ ID NO: 19793 - RNA, 20 nt, synthetic construct
  source 1..20: mol_type = other RNA
ggcacgaaaagacagcagag

SEQ ID NO: 19794 - RNA, 20 nt, synthetic construct
  source 1..20: mol_type = other RNA
gtgtccccaagctgctgccc

SEQ ID NO: 19795 - RNA, 20 nt, synthetic construct
  source 1..20: mol_type = other RNA
ggctcctgggcagcagcttg

SEQ ID NO: 19796 - RNA, 20 nt, synthetic construct
  source 1..20: mol_type = other RNA
gctgctgcccaggagcccaa

SEQ ID NO: 19797 - RNA, 20 nt, synthetic construct
  source 1..20: mol_type = other RNA
tgggctcctgggcagcagct

SEQ ID NO: 19798 - RNA, 20 nt, synthetic construct
  source 1..20: mol_type = other RNA
gctgcccaggagcccaaggg

SEQ ID NO: 19799 - RNA, 20 nt, synthetic construct
  source 1..20: mol_type = other RNA
ctgcccaggagcccaagggt

SEQ ID NO: 19800 - RNA, 20 nt, synthetic construct
  source 1..20: mol_type = other RNA
ctgcccacccttgggctcct

SEQ ID NO: 19801 - RNA, 20 nt, synthetic construct
  source 1..20: mol_type = other RNA
actgcccacccttgggctcc

SEQ ID NO: 19802 - RNA, 20 nt, synthetic construct
  source 1..20: mol_type = other RNA
gacaaagactgcccaccctt

SEQ ID NO: 19803 - RNA, 20 nt, synthetic construct
  source 1..20: mol_type = other RNA
agacaaagactgcccaccct

SEQ ID NO: 19804 - RNA, 20 nt, synthetic construct
  source 1..20: mol_type = other RNA
gggcagtctttgtctgacac

SEQ ID NO: 19805 - RNA, 20 nt, synthetic construct
  source 1..20: mol_type = other RNA
aaccccttcacttcacattt

SEQ ID NO: 19806 - RNA, 20 nt, synthetic construct
  source 1..20: mol_type = other RNA
accccttcacttcacattta

SEQ ID NO: 19807 - RNA, 20 nt, synthetic construct
  source 1..20: mol_type = other RNA
ccccttcacttcacatttag

SEQ ID NO: 19808 - RNA, 20 nt, synthetic construct
  source 1..20: mol_type = other RNA
cccctaaatgtgaagtgaag

SEQ ID NO: 19809 - RNA, 20 nt, synthetic construct
  source 1..20: mol_type = other RNA
tcccctaaatgtgaagtgaa

SEQ ID NO: 19810 - RNA, 20 nt, synthetic construct
  source 1..20: mol_type = other RNA
acttcacatttaggggattg

SEQ ID NO: 19811 - RNA, 20 nt, synthetic construct
  source 1..20: mol_type = other RNA
tttaggggattgaggcctag

SEQ ID NO: 19812 - RNA, 20 nt, synthetic construct
  source 1..20: mol_type = other RNA
ggattgaggcctagtggagc

SEQ ID NO: 19813 - RNA, 20 nt, synthetic construct
  source 1..20: mol_type = other RNA
gattgaggcctagtggagca

SEQ ID NO: 19814 - RNA, 20 nt, synthetic construct
  source 1..20: mol_type = other RNA
gtggagcagggactcaccca

SEQ ID NO: 19815 - RNA, 20 nt, synthetic construct
  source 1..20: mol_type = other RNA
gggtgagtccctgctccact

SEQ ID NO: 19816 - RNA, 20 nt, synthetic construct
  source 1..20: mol_type = other RNA
ggactcacccacggccacac

SEQ ID NO: 19817 - RNA, 20 nt, synthetic construct
  source 1..20: mol_type = other RNA
gactcacccacggccacaca

SEQ ID NO: 19818 - RNA, 20 nt, synthetic construct
  source 1..20: mol_type = other RNA
actcacccacggccacacag

SEQ ID NO: 19819 - RNA, 20 nt, synthetic construct
  source 1..20: mol_type = other RNA
ctcacccacggccacacagg

SEQ ID NO: 19820 - RNA, 20 nt, synthetic construct
  source 1..20: mol_type = other RNA
ctgaccccctgtgtggccgt

SEQ ID NO: 19821 - RNA, 20 nt, synthetic construct
  source 1..20: mol_type = other RNA
tctgaccccctgtgtggccg

SEQ ID NO: 19822 - RNA, 20 nt, synthetic construct
  source 1..20: mol_type = other RNA
agtaattctgaccccctgtg

SEQ ID NO: 19823 - RNA, 20 nt, synthetic construct
  source 1..20: mol_type = other RNA
gggggtcagaattactgttg

SEQ ID NO: 19824 - RNA, 20 nt, synthetic construct
  source 1..20: mol_type = other RNA
actgaaacaattctggattc

SEQ ID NO: 19825 - RNA, 20 nt, synthetic construct
  source 1..20: mol_type = other RNA
gaattgtttcagttccaacc

SEQ ID NO: 19826 - RNA, 20 nt, synthetic construct
  source 1..20: mol_type = other RNA
ggttggaactgaaacaattc

SEQ ID NO: 19827 - RNA, 20 nt, synthetic construct
  source 1..20: mol_type = other RNA
tgtttcagttccaaccagga

SEQ ID NO: 19828 - RNA, 20 nt, synthetic construct
  source 1..20: mol_type = other RNA
gtttcagttccaaccaggaa

SEQ ID NO: 19829 - RNA, 20 nt, synthetic construct
  source 1..20: mol_type = other RNA
tttcagttccaaccaggaag

SEQ ID NO: 19830 - RNA, 20 nt, synthetic construct
  source 1..20: mol_type = other RNA
gaaacaaaccccttcctggt

SEQ ID NO: 19831 - RNA, 20 nt, synthetic construct
  source 1..20: mol_type = other RNA
ttgggaaacaaaccccttcc

SEQ ID NO: 19832 - RNA, 20 nt, synthetic construct
  source 1..20: mol_type = other RNA
gtggggtagggacaggtttt

SEQ ID NO: 19833 - RNA, 20 nt, synthetic construct
  source 1..20: mol_type = other RNA
ggtggggtagggacaggttt

SEQ ID NO: 19834 - RNA, 20 nt, synthetic construct
  source 1..20: mol_type = other RNA
tccctaccccaccccttctt

SEQ ID NO: 19835 - RNA, 20 nt, synthetic construct
  source 1..20: mol_type = other RNA
agaaggggtggggtagggac

SEQ ID NO: 19836 - RNA, 20 nt, synthetic construct
  source 1..20: mol_type = other RNA
taccccaccccttctttggc

SEQ ID NO: 19837 - RNA, 20 nt, synthetic construct
  source 1..20: mol_type = other RNA
gccaaagaaggggtggggta

SEQ ID NO: 19838 - RNA, 20 nt, synthetic construct
  source 1..20: mol_type = other RNA
cccaccccttctttggcagg

SEQ ID NO: 19839 - RNA, 20 nt, synthetic construct
  source 1..20: mol_type = other RNA
cgcctgccaaagaaggggtg

SEQ ID NO: 19840 - RNA, 20 nt, synthetic construct
  source 1..20: mol_type = other RNA
ccgcctgccaaagaaggggt

SEQ ID NO: 19841 - RNA, 20 nt, synthetic construct
  source 1..20: mol_type = other RNA
tccgcctgccaaagaagggg

SEQ ID NO: 19842 - RNA, 20 nt, synthetic construct
  source 1..20: mol_type = other RNA
tactccgcctgccaaagaag

SEQ ID NO: 19843 - RNA, 20 nt, synthetic construct
  source 1..20: mol_type = other RNA
ctactccgcctgccaaagaa

SEQ ID NO: 19844 - RNA, 20 nt, synthetic construct
  source 1..20: mol_type = other RNA
gctactccgcctgccaaaga

SEQ ID NO: 19845 - RNA, 20 nt, synthetic construct
  source 1..20: mol_type = other RNA
gcggagtagctgtcgccctc

SEQ ID NO: 19846 - RNA, 20 nt, synthetic construct
  source 1..20: mol_type = other RNA
cggagtagctgtcgccctca

SEQ ID NO: 19847 - RNA, 20 nt, synthetic construct
  source 1..20: mol_type = other RNA
agtagctgtcgccctcaggg

SEQ ID NO: 19848 - RNA, 20 nt, synthetic construct
  source 1..20: mol_type = other RNA
agggtggcccagagcagtgc

SEQ ID NO: 19849 - RNA, 20 nt, synthetic construct
  source 1..20: mol_type = other RNA
gggtggcccagagcagtgct

SEQ ID NO: 19850 - RNA, 20 nt, synthetic construct
  source 1..20: mol_type = other RNA
ggtggcccagagcagtgctg

SEQ ID NO: 19851 - RNA, 20 nt, synthetic construct
  source 1..20: mol_type = other RNA
gtggcccagagcagtgctgg

SEQ ID NO: 19852 - RNA, 20 nt, synthetic construct
  source 1..20: mol_type = other RNA
tctacccccagcactgctct

SEQ ID NO: 19853 - RNA, 20 nt, synthetic construct
  source 1..20: mol_type = other RNA
ctctacccccagcactgctc

SEQ ID NO: 19854 - RNA, 20 nt, synthetic construct
  source 1..20: mol_type = other RNA
agtgctgggggtagagatga

SEQ ID NO: 19855 - RNA, 20 nt, synthetic construct
  source 1..20: mol_type = other RNA
ttgtgaagacactgccaaga

SEQ ID NO: 19856 - RNA, 20 nt, synthetic construct
  source 1..20: mol_type = other RNA
tgtgaagacactgccaagaa

SEQ ID NO: 19857 - RNA, 20 nt, synthetic construct
  source 1..20: mol_type = other RNA
gtgaagacactgccaagaag

SEQ ID NO: 19858 - RNA, 20 nt, synthetic construct
  source 1..20: mol_type = other RNA
ttcttggcagtgtcttcaca

SEQ ID NO: 19859 - RNA, 20 nt, synthetic construct
  source 1..20: mol_type = other RNA
aagacactgccaagaagggg

SEQ ID NO: 19860 - RNA, 20 nt, synthetic construct
  source 1..20: mol_type = other RNA
agacactgccaagaaggggt

SEQ ID NO: 19861 - RNA, 20 nt, synthetic construct
  source 1..20: mol_type = other RNA
gacactgccaagaaggggtg

SEQ ID NO: 19862 - RNA, 20 nt, synthetic construct
  source 1..20: mol_type = other RNA
gaagttgccccaccccttct

SEQ ID NO: 19863 - RNA, 20 nt, synthetic construct
  source 1..20: mol_type = other RNA
ggggtggggcaacttccaag

SEQ ID NO: 19864 - RNA, 20 nt, synthetic construct
  source 1..20: mol_type = other RNA
cttcttggtgctcttcctct

SEQ ID NO: 19865 - RNA, 20 nt, synthetic construct
  source 1..20: mol_type = other RNA
caagaagcccaaaccccaga

SEQ ID NO: 19866 - RNA, 20 nt, synthetic construct
  source 1..20: mol_type = other RNA
cgtctggggtttgggcttct

SEQ ID NO: 19867 - RNA, 20 nt, synthetic construct
  source 1..20: mol_type = other RNA
ttggtttccgtctggggttt

SEQ ID NO: 19868 - RNA, 20 nt, synthetic construct
  source 1..20: mol_type = other RNA
tttggtttccgtctggggtt

SEQ ID NO: 19869 - RNA, 20 nt, synthetic construct
  source 1..20: mol_type = other RNA
atacatttggtttccgtctg

SEQ ID NO: 19870 - RNA, 20 nt, synthetic construct
  source 1..20: mol_type = other RNA
aatacatttggtttccgtct

SEQ ID NO: 19871 - RNA, 20 nt, synthetic construct
  source 1..20: mol_type = other RNA
aaatacatttggtttccgtc

SEQ ID NO: 19872 - RNA, 20 nt, synthetic construct
  source 1..20: mol_type = other RNA
ggaaaccaaatgtattttct

SEQ ID NO: 19873 - RNA, 20 nt, synthetic construct
  source 1..20: mol_type = other RNA
tgtattttctgggccctgag

SEQ ID NO: 19874 - RNA, 20 nt, synthetic construct
  source 1..20: mol_type = other RNA
ctgggccctgagaggatatt

SEQ ID NO: 19875 - RNA, 20 nt, synthetic construct
  source 1..20: mol_type = other RNA
tgagaggatatttggaacaa

SEQ ID NO: 19876 - RNA, 20 nt, synthetic construct
  source 1..20: mol_type = other RNA
ttgttccaaatatcctctca

SEQ ID NO: 19877 - RNA, 20 nt, synthetic construct
  source 1..20: mol_type = other RNA
gaggatatttggaacaatgg

SEQ ID NO: 19878 - RNA, 20 nt, synthetic construct
  source 1..20: mol_type = other RNA
gatatttggaacaatggagg

SEQ ID NO: 19879 - RNA, 20 nt, synthetic construct
  source 1..20: mol_type = other RNA
atatttggaacaatggaggt

SEQ ID NO: 19880 - RNA, 20 nt, synthetic construct
  source 1..20: mol_type = other RNA
ggaacaatggaggtgggatg

SEQ ID NO: 19881 - RNA, 20 nt, synthetic construct
  source 1..20: mol_type = other RNA
gaacaatggaggtgggatga

SEQ ID NO: 19882 - RNA, 20 nt, synthetic construct
  source 1..20: mol_type = other RNA
tgggatgagggaagttaaaa

SEQ ID NO: 19883 - RNA, 20 nt, synthetic construct
  source 1..20: mol_type = other RNA
gggatgagggaagttaaaaa

SEQ ID NO: 19884 - RNA, 20 nt, synthetic construct
  source 1..20: mol_type = other RNA
tccttagaaaaaaaaaatac

SEQ ID NO: 19885 - RNA, 20 nt, synthetic construct
  source 1..20: mol_type = other RNA
gcctgtattttttttttcta

SEQ ID NO: 19886 - RNA, 20 nt, synthetic construct
  source 1..20: mol_type = other RNA
tttgacttttgtttctctga

SEQ ID NO: 19887 - RNA, 20 nt, synthetic construct
  source 1..20: mol_type = other RNA
atgtttgtgtaactttctga

SEQ ID NO: 19888 - RNA, 20 nt, synthetic construct
  source 1..20: mol_type = other RNA
ttgtgtaactttctgaaggc

SEQ ID NO: 19889 - RNA, 20 nt, synthetic construct
  source 1..20: mol_type = other RNA
gacaagcttcacagagtgct

SEQ ID NO: 19890 - RNA, 20 nt, synthetic construct
  source 1..20: mol_type = other RNA
tgacaagcttcacagagtgc

SEQ ID NO: 19891 - RNA, 20 nt, synthetic construct
  source 1..20: mol_type = other RNA
cagagtctgctctgttgccc

SEQ ID NO: 19892 - RNA, 20 nt, synthetic construct
  source 1..20: mol_type = other RNA
gtctgctctgttgcccaggc

SEQ ID NO: 19893 - RNA, 20 nt, synthetic construct
  source 1..20: mol_type = other RNA
ttgcccaggctggagtgcag

SEQ ID NO: 19894 - RNA, 20 nt, synthetic construct
  source 1..20: mol_type = other RNA
gcgccactgcactccagcct

SEQ ID NO: 19895 - RNA, 20 nt, synthetic construct
  source 1..20: mol_type = other RNA
cgcgccactgcactccagcc

SEQ ID NO: 19896 - RNA, 20 nt, synthetic construct
  source 1..20: mol_type = other RNA
ggagtgcagtggcgcgatct

SEQ ID NO: 19897 - RNA, 20 nt, synthetic construct
  source 1..20: mol_type = other RNA
tcactgcagcctccatctcc

SEQ ID NO: 19898 - RNA, 20 nt, synthetic construct
  source 1..20: mol_type = other RNA
cactgcagcctccatctccc

SEQ ID NO: 19899 - RNA, 20 nt, synthetic construct
  source 1..20: mol_type = other RNA
cgcttgaacccgggagatgg

SEQ ID NO: 19900 - RNA, 20 nt, synthetic construct
  source 1..20: mol_type = other RNA
aatcgcttgaacccgggaga

SEQ ID NO: 19901 - RNA, 20 nt, synthetic construct
  source 1..20: mol_type = other RNA
caggagaatcgcttgaaccc

SEQ ID NO: 19902 - RNA, 20 nt, synthetic construct
  source 1..20: mol_type = other RNA
gcaggagaatcgcttgaacc

SEQ ID NO: 19903 - RNA, 20 nt, synthetic construct
  source 1..20: mol_type = other RNA
gcctcggcctcccgaatagc

SEQ ID NO: 19904 - RNA, 20 nt, synthetic construct
  source 1..20: mol_type = other RNA
cctcggcctcccgaatagct

SEQ ID NO: 19905 - RNA, 20 nt, synthetic construct
  source 1..20: mol_type = other RNA
gctattcgggaggccgaggc

SEQ ID NO: 19906 - RNA, 20 nt, synthetic construct
  source 1..20: mol_type = other RNA
cccagctattcgggaggccg

SEQ ID NO: 19907 - RNA, 20 nt, synthetic construct
  source 1..20: mol_type = other RNA
tcccgaatagctgggattac

SEQ ID NO: 19908 - RNA, 20 nt, synthetic construct
  source 1..20: mol_type = other RNA
agtaatcccagctattcggg

SEQ ID NO: 19909 - RNA, 20 nt, synthetic construct
  source 1..20: mol_type = other RNA
accagtaatcccagctattc

SEQ ID NO: 19910 - RNA, 20 nt, synthetic construct
  source 1..20: mol_type = other RNA
caccagtaatcccagctatt

SEQ ID NO: 19911 - RNA, 20 nt, synthetic construct
  source 1..20: mol_type = other RNA
aaaaatttagctgggtatgg

SEQ ID NO: 19912 - RNA, 20 nt, synthetic construct
  source 1..20: mol_type = other RNA
aaaaaaaatttagctgggta

SEQ ID NO: 19913 - RNA, 20 nt, synthetic construct
  source 1..20: mol_type = other RNA
aatacaaaaaaaatttagct

SEQ ID NO: 19914 - RNA, 20 nt, synthetic construct
  source 1..20: mol_type = other RNA
aaatacaaaaaaaatttagc

SEQ ID NO: 19915 - RNA, 20 nt, synthetic construct
  source 1..20: mol_type = other RNA
ttttgtatttttagtagaga

SEQ ID NO: 19916 - RNA, 20 nt, synthetic construct
  source 1..20: mol_type = other RNA
tttgtatttttagtagagac

SEQ ID NO: 19917 - RNA, 20 nt, synthetic construct
  source 1..20: mol_type = other RNA
ttgtatttttagtagagacg

SEQ ID NO: 19918 - RNA, 20 nt, synthetic construct
  source 1..20: mol_type = other RNA
ggggtttcaccatattgacc

SEQ ID NO: 19919 - RNA, 20 nt, synthetic construct
  source 1..20: mol_type = other RNA
tttcaccatattgaccaggc

SEQ ID NO: 19920 - RNA, 20 nt, synthetic construct
  source 1..20: mol_type = other RNA
cgagaccagcctggtcaata

SEQ ID NO: 19921 - RNA, 20 nt, synthetic construct
  source 1..20: mol_type = other RNA
tcaggagttcgagaccagcc

SEQ ID NO: 19922 - RNA, 20 nt, synthetic construct
  source 1..20: mol_type = other RNA
ggtctcgaactcctgacctc

SEQ ID NO: 19923 - RNA, 20 nt, synthetic construct
  source 1..20: mol_type = other RNA
caggcagatcacctgaggtc

SEQ ID NO: 19924 - RNA, 20 nt, synthetic construct
  source 1..20: mol_type = other RNA
ctcaggtgatctgcctgctt

SEQ ID NO: 19925 - RNA, 20 nt, synthetic construct
  source 1..20: mol_type = other RNA
caaagcaggcagatcacctg

SEQ ID NO: 19926 - RNA, 20 nt, synthetic construct
  source 1..20: mol_type = other RNA
gctttggcctcccaaagtgc

SEQ ID NO: 19927 - RNA, 20 nt, synthetic construct
  source 1..20: mol_type = other RNA
ctttggcctcccaaagtgct

SEQ ID NO: 19928 - RNA, 20 nt, synthetic construct
  source 1..20: mol_type = other RNA
gcactttgggaggccaaagc

SEQ ID NO: 19929 - RNA, 20 nt, synthetic construct
  source 1..20: mol_type = other RNA
tcccaaagtgctgggattgc

SEQ ID NO: 19930 - RNA, 20 nt, synthetic construct
  source 1..20: mol_type = other RNA
tgcaatcccagcactttggg

SEQ ID NO: 19931 - RNA, 20 nt, synthetic construct
  source 1..20: mol_type = other RNA
gcctgcaatcccagcacttt

SEQ ID NO: 19932 - RNA, 20 nt, synthetic construct
  source 1..20: mol_type = other RNA
tgcctgcaatcccagcactt

SEQ ID NO: 19933 - RNA, 20 nt, synthetic construct
  source 1..20: mol_type = other RNA
caggcatgagctaccacgcc

SEQ ID NO: 19934 - RNA, 20 nt, synthetic construct
  source 1..20: mol_type = other RNA
agctaccacgcctggccatt

SEQ ID NO: 19935 - RNA, 20 nt, synthetic construct
  source 1..20: mol_type = other RNA
cagcacctaatggccaggcg

SEQ ID NO: 19936 - RNA, 20 nt, synthetic construct
  source 1..20: mol_type = other RNA
aaaaacagcacctaatggcc

SEQ ID NO: 19937 - RNA, 20 nt, synthetic construct
  source 1..20: mol_type = other RNA
tctataaaaacagcacctaa

SEQ ID NO: 19938 - RNA, 20 nt, synthetic construct
  source 1..20: mol_type = other RNA
ggtgctgtttttatagattc

SEQ ID NO: 19939 - RNA, 20 nt, synthetic construct
  source 1..20: mol_type = other RNA
gtgctgtttttatagattca

SEQ ID NO: 19940 - RNA, 20 nt, synthetic construct
  source 1..20: mol_type = other RNA
tttttatagattcagggctt

SEQ ID NO: 19941 - RNA, 20 nt, synthetic construct
  source 1..20: mol_type = other RNA
tagattcagggctttggagc

SEQ ID NO: 19942 - RNA, 20 nt, synthetic construct
  source 1..20: mol_type = other RNA
agattcagggctttggagct

SEQ ID NO: 19943 - RNA, 20 nt, synthetic construct
  source 1..20: mol_type = other RNA
tcagggctttggagctggga

SEQ ID NO: 19944 - RNA, 20 nt, synthetic construct
  source 1..20: mol_type = other RNA
tagtctcctcactttatagt

SEQ ID NO: 19945 - RNA, 20 nt, synthetic construct
  source 1..20: mol_type = other RNA
tcactttatagttggtgaaa

SEQ ID NO: 19946 - RNA, 20 nt, synthetic construct
  source 1..20: mol_type = other RNA
atttcaccaactataaagtg

SEQ ID NO: 19947 - RNA, 20 nt, synthetic construct
  source 1..20: mol_type = other RNA
ttggtgaaatggaggctgag

SEQ ID NO: 19948 - RNA, 20 nt, synthetic construct
  source 1..20: mol_type = other RNA
gtgaaatggaggctgagagg

SEQ ID NO: 19949 - RNA, 20 nt, synthetic construct
  source 1..20: mol_type = other RNA
tgaaatggaggctgagaggt

SEQ ID NO: 19950 - RNA, 20 nt, synthetic construct
  source 1..20: mol_type = other RNA
gaaatggaggctgagaggtg

SEQ ID NO: 19951 - RNA, 20 nt, synthetic construct
  source 1..20: mol_type = other RNA
aaatggaggctgagaggtgg

SEQ ID NO: 19952 - RNA, 20 nt, synthetic construct
  source 1..20: mol_type = other RNA
aatggaggctgagaggtggg

SEQ ID NO: 19953 - RNA, 20 nt, synthetic construct
  source 1..20: mol_type = other RNA
agaggtggggggcctgcttg

SEQ ID NO: 19954 - RNA, 20 nt, synthetic construct
  source 1..20: mol_type = other RNA
ctgcttgaggtcacacagtg

SEQ ID NO: 19955 - RNA, 20 nt, synthetic construct
  source 1..20: mol_type = other RNA
ctcactgtgtgacctcaagc

SEQ ID NO: 19956 - RNA, 20 nt, synthetic construct
  source 1..20: mol_type = other RNA
gtcacacagtgaggcagccg

SEQ ID NO: 19957 - RNA, 20 nt, synthetic construct
  source 1..20: mol_type = other RNA
cagtgaggcagccgaggtct

SEQ ID NO: 19958 - RNA, 20 nt, synthetic construct
  source 1..20: mol_type = other RNA
cataggaagatccaagacct

SEQ ID NO: 19959 - RNA, 20 nt, synthetic construct
  source 1..20: mol_type = other RNA
atcttcctatgtgttgcaag

SEQ ID NO: 19960 - RNA, 20 nt, synthetic construct
  source 1..20: mol_type = other RNA
gacagcctcttgcaacacat

SEQ ID NO: 19961 - RNA, 20 nt, synthetic construct
  source 1..20: mol_type = other RNA
catcttgacttaccacctcc

SEQ ID NO: 19962 - RNA, 20 nt, synthetic construct
  source 1..20: mol_type = other RNA
atcttgacttaccacctcct

SEQ ID NO: 19963 - RNA, 20 nt, synthetic construct
  source 1..20: mol_type = other RNA
caggaggtggtaagtcaaga

SEQ ID NO: 19964 - RNA, 20 nt, synthetic construct
  source 1..20: mol_type = other RNA
acttaccacctcctgggacc

SEQ ID NO: 19965 - RNA, 20 nt, synthetic construct
  source 1..20: mol_type = other RNA
accacctcctgggacctggc

SEQ ID NO: 19966 - RNA, 20 nt, synthetic construct
  source 1..20: mol_type = other RNA
ctcctgggacctggctggca

SEQ ID NO: 19967 - RNA, 20 nt, synthetic construct
  source 1..20: mol_type = other RNA
tcctgggacctggctggcat

SEQ ID NO: 19968 - RNA, 20 nt, synthetic construct
  source 1..20: mol_type = other RNA
cctgggacctggctggcatg

SEQ ID NO: 19969 - RNA, 20 nt, synthetic construct
  source 1..20: mol_type = other RNA
ctgggacctggctggcatgg

SEQ ID NO: 19970 - RNA, 20 nt, synthetic construct
  source 1..20: mol_type = other RNA
catgccagccaggtcccagg

SEQ ID NO: 19971 - RNA, 20 nt, synthetic construct
  source 1..20: mol_type = other RNA
ccccatgccagccaggtccc

SEQ ID NO: 19972 - RNA, 20 nt, synthetic construct
  source 1..20: mol_type = other RNA
acctggctggcatgggggct

SEQ ID NO: 19973 - RNA, 20 nt, synthetic construct
  source 1..20: mol_type = other RNA
tggctggcatgggggctggg

SEQ ID NO: 19974 - RNA, 20 nt, synthetic construct
  source 1..20: mol_type = other RNA
gcccagcccccatgccagcc

SEQ ID NO: 19975 - RNA, 20 nt, synthetic construct
  source 1..20: mol_type = other RNA
gggctgggcggtcactgatg

SEQ ID NO: 19976 - RNA, 20 nt, synthetic construct
  source 1..20: mol_type = other RNA
ggctgggcggtcactgatga

SEQ ID NO: 19977 - RNA, 20 nt, synthetic construct
  source 1..20: mol_type = other RNA
gctgggcggtcactgatgag

SEQ ID NO: 19978 - RNA, 20 nt, synthetic construct
  source 1..20: mol_type = other RNA
ttcaaaatgctcattgctgc

SEQ ID NO: 19979 - RNA, 20 nt, synthetic construct
  source 1..20: mol_type = other RNA
tcaaaatgctcattgctgct

SEQ ID NO: 19980 - RNA, 20 nt, synthetic construct
  source 1..20: mol_type = other RNA
caaaatgctcattgctgctg

SEQ ID NO: 19981 - RNA, 20 nt, synthetic construct
  source 1..20: mol_type = other RNA
agcagcaatgagcattttga

SEQ ID NO: 19982 - RNA, 20 nt, synthetic construct
  source 1..20: mol_type = other RNA
tgctcattgctgctggggat

SEQ ID NO: 19983 - RNA, 20 nt, synthetic construct
  source 1..20: mol_type = other RNA
ttgctgctggggataggata

SEQ ID NO: 19984 - RNA, 20 nt, synthetic construct
  source 1..20: mol_type = other RNA
gctggggataggataaggcc

SEQ ID NO: 19985 - RNA, 20 nt, synthetic construct
  source 1..20: mol_type = other RNA
ggataggataaggccaggtc

SEQ ID NO: 19986 - RNA, 20 nt, synthetic construct
  source 1..20: mol_type = other RNA
gataaggccaggtctggtct

SEQ ID NO: 19987 - RNA, 20 nt, synthetic construct
  source 1..20: mol_type = other RNA
ataaggccaggtctggtctt

SEQ ID NO: 19988 - RNA, 20 nt, synthetic construct
  source 1..20: mol_type = other RNA
atcttgcccaagaccagacc

SEQ ID NO: 19989 - RNA, 20 nt, synthetic construct
  source 1..20: mol_type = other RNA
cttgggcaagatgagcccac

SEQ ID NO: 19990 - RNA, 20 nt, synthetic construct
  source 1..20: mol_type = other RNA
gggcaagatgagcccactgg

SEQ ID NO: 19991 - RNA, 20 nt, synthetic construct
  source 1..20: mol_type = other RNA
ggcaagatgagcccactggt

SEQ ID NO: 19992 - RNA, 20 nt, synthetic construct
  source 1..20: mol_type = other RNA
gcaagatgagcccactggtg

SEQ ID NO: 19993 - RNA, 20 nt, synthetic construct
  source 1..20: mol_type = other RNA
tgagcccactggtggggaga

SEQ ID NO: 19994 - RNA, 20 nt, synthetic construct
  source 1..20: mol_type = other RNA
tcagccttctccccaccagt

SEQ ID NO: 19995 - RNA, 20 nt, synthetic construct
  source 1..20: mol_type = other RNA
ctcagccttctccccaccag

SEQ ID NO: 19996 - RNA, 20 nt, synthetic construct
  source 1..20: mol_type = other RNA
gaaggctgagatggtacacc

SEQ ID NO: 19997 - RNA, 20 nt, synthetic construct
  source 1..20: mol_type = other RNA
tggatgagggtggcattacc

SEQ ID NO: 19998 - RNA, 20 nt, synthetic construct
  source 1..20: mol_type = other RNA
gccaccctcatccagatgcc

SEQ ID NO: 19999 - RNA, 20 nt, synthetic construct
  source 1..20: mol_type = other RNA
gcctggcatctggatgaggg

SEQ ID NO: 20000 - RNA, 20 nt, synthetic construct
  source 1..20: mol_type = other RNA
tgggcctggcatctggatga

SEQ ID NO: 20001 - RNA, 20 nt, synthetic construct
  source 1..20: mol_type = other RNA
ctgggcctggcatctggatg

SEQ ID NO: 20002 - RNA, 20 nt, synthetic construct
  source 1..20: mol_type = other RNA
gcacagctgggcctggcatc

SEQ ID NO: 20003 - RNA, 20 nt, synthetic construct
  source 1..20: mol_type = other RNA
agacggtgcacagctgggcc

SEQ ID NO: 20004 - RNA, 20 nt, synthetic construct
  source 1..20: mol_type = other RNA
tgggcagacggtgcacagct

SEQ ID NO: 20005 - RNA, 20 nt, synthetic construct
  source 1..20: mol_type = other RNA
ctgggcagacggtgcacagc

SEQ ID NO: 20006 - RNA, 20 nt, synthetic construct
  source 1..20: mol_type = other RNA
tgcaccgtctgcccagcagc

SEQ ID NO: 20007 - RNA, 20 nt, synthetic construct
  source 1..20: mol_type = other RNA
gcaccgtctgcccagcagct

SEQ ID NO: 20008 - RNA, 20 nt, synthetic construct
  source 1..20: mol_type = other RNA
gctcccagctgctgggcaga

SEQ ID NO: 20009 - RNA, 20 nt, synthetic construct
  source 1..20: mol_type = other RNA
actcacagctcccagctgct

SEQ ID NO: 20010 - RNA, 20 nt, synthetic construct
  source 1..20: mol_type = other RNA
gactcacagctcccagctgc

SEQ ID NO: 20011 - RNA, 20 nt, synthetic construct
  source 1..20: mol_type = other RNA
gagctgtgagtcacacccag

SEQ ID NO: 20012 - RNA, 20 nt, synthetic construct
  source 1..20: mol_type = other RNA
gtcacacccagtggatacag

SEQ ID NO: 20013 - RNA, 20 nt, synthetic construct
  source 1..20: mol_type = other RNA
cccagtggatacagaggcgc

SEQ ID NO: 20014 - RNA, 20 nt, synthetic construct
  source 1..20: mol_type = other RNA
cctgcgcctctgtatccact

SEQ ID NO: 20015 - RNA, 20 nt, synthetic construct
  source 1..20: mol_type = other RNA
gcctgcgcctctgtatccac

SEQ ID NO: 20016 - RNA, 20 nt, synthetic construct
  source 1..20: mol_type = other RNA
gaatgaatcacggcacacaa

SEQ ID NO: 20017 - RNA, 20 nt, synthetic construct
  source 1..20: mol_type = other RNA
cgtgattcattctgttctcc

SEQ ID NO: 20018 - RNA, 20 nt, synthetic construct
  source 1..20: mol_type = other RNA
cgggagaacagaatgaatca

SEQ ID NO: 20019 - RNA, 20 nt, synthetic construct
  source 1..20: mol_type = other RNA
ttctgttctcccggccccga

SEQ ID NO: 20020 - RNA, 20 nt, synthetic construct
  source 1..20: mol_type = other RNA
tctgttctcccggccccgaa

SEQ ID NO: 20021 - RNA, 20 nt, synthetic construct
  source 1..20: mol_type = other RNA
ccggccccgaagggatgacg

SEQ ID NO: 20022 - RNA, 20 nt, synthetic construct
  source 1..20: mol_type = other RNA
ctcgtcatcccttcggggcc

SEQ ID NO: 20023 - RNA, 20 nt, synthetic construct
  source 1..20: mol_type = other RNA
cctcgtcatcccttcggggc

SEQ ID NO: 20024 - RNA, 20 nt, synthetic construct
  source 1..20: mol_type = other RNA
agggcctcgtcatcccttcg

SEQ ID NO: 20025 - RNA, 20 nt, synthetic construct
  source 1..20: mol_type = other RNA
cagggcctcgtcatcccttc

SEQ ID NO: 20026 - RNA, 20 nt, synthetic construct
  source 1..20: mol_type = other RNA
tcagggcctcgtcatccctt

SEQ ID NO: 20027 - RNA, 20 nt, synthetic construct
  source 1..20: mol_type = other RNA
tgggcatggatcggtgctca

SEQ ID NO: 20028 - RNA, 20 nt, synthetic construct
  source 1..20: mol_type = other RNA
gtgggcatggatcggtgctc

SEQ ID NO: 20029 - RNA, 20 nt, synthetic construct
  source 1..20: mol_type = other RNA
ccgatccatgcccacgcctg

SEQ ID NO: 20030 - RNA, 20 nt, synthetic construct
  source 1..20: mol_type = other RNA
ccacaggcgtgggcatggat

SEQ ID NO: 20031 - RNA, 20 nt, synthetic construct
  source 1..20: mol_type = other RNA
ttcatccacaggcgtgggca

SEQ ID NO: 20032 - RNA, 20 nt, synthetic construct
  source 1..20: mol_type = other RNA
cagctttcatccacaggcgt

SEQ ID NO: 20033 - RNA, 20 nt, synthetic construct
  source 1..20: mol_type = other RNA
tcagctttcatccacaggcg

SEQ ID NO: 20034 - RNA, 20 nt, synthetic construct
  source 1..20: mol_type = other RNA
tgtggatgaaagctgatatg

SEQ ID NO: 20035 - RNA, 20 nt, synthetic construct
  source 1..20: mol_type = other RNA
ggatgaaagctgatatgagg

SEQ ID NO: 20036 - RNA, 20 nt, synthetic construct
  source 1..20: mol_type = other RNA
aagctgatatgaggaggccc

SEQ ID NO: 20037 - RNA, 20 nt, synthetic construct
  source 1..20: mol_type = other RNA
agctgatatgaggaggccca

SEQ ID NO: 20038 - RNA, 20 nt, synthetic construct
  source 1..20: mol_type = other RNA
gctgatatgaggaggcccag

SEQ ID NO: 20039 - RNA, 20 nt, synthetic construct
  source 1..20: mol_type = other RNA
gaggaggcccaggggacctg

SEQ ID NO: 20040 - RNA, 20 nt, synthetic construct
  source 1..20: mol_type = other RNA
aggaggcccaggggacctga

SEQ ID NO: 20041 - RNA, 20 nt, synthetic construct
  source 1..20: mol_type = other RNA
cccaggggacctgagggagt

SEQ ID NO: 20042 - RNA, 20 nt, synthetic construct
  source 1..20: mol_type = other RNA
ccgactccctcaggtcccct

SEQ ID NO: 20043 - RNA, 20 nt, synthetic construct
  source 1..20: mol_type = other RNA
gccgactccctcaggtcccc

SEQ ID NO: 20044 - RNA, 20 nt, synthetic construct
  source 1..20: mol_type = other RNA
cagagggagccgactccctc

SEQ ID NO: 20045 - RNA, 20 nt, synthetic construct
  source 1..20: mol_type = other RNA
aagagacaggaggtagcaga

SEQ ID NO: 20046 - RNA, 20 nt, synthetic construct
  source 1..20: mol_type = other RNA
caagagacaggaggtagcag

SEQ ID NO: 20047 - RNA, 20 nt, synthetic construct
  source 1..20: mol_type = other RNA
caggatactcaagagacagg

SEQ ID NO: 20048 - RNA, 20 nt, synthetic construct
  source 1..20: mol_type = other RNA
tcacaggatactcaagagac

SEQ ID NO: 20049 - RNA, 20 nt, synthetic construct
  source 1..20: mol_type = other RNA
aatggacaggtcacgatcac

SEQ ID NO: 20050 - RNA, 20 nt, synthetic construct
  source 1..20: mol_type = other RNA
ctgtccattcccaccagtgc

SEQ ID NO: 20051 - RNA, 20 nt, synthetic construct
  source 1..20: mol_type = other RNA
tgtccattcccaccagtgca

SEQ ID NO: 20052 - RNA, 20 nt, synthetic construct
  source 1..20: mol_type = other RNA
gtccattcccaccagtgcag

SEQ ID NO: 20053 - RNA, 20 nt, synthetic construct
  source 1..20: mol_type = other RNA
ctgcactggtgggaatggac

SEQ ID NO: 20054 - RNA, 20 nt, synthetic construct
  source 1..20: mol_type = other RNA
gacccctgcactggtgggaa

SEQ ID NO: 20055 - RNA, 20 nt, synthetic construct
  source 1..20: mol_type = other RNA
tcatggacccctgcactggt

SEQ ID NO: 20056 - RNA, 20 nt, synthetic construct
  source 1..20: mol_type = other RNA
ctcatggacccctgcactgg

SEQ ID NO: 20057 - RNA, 20 nt, synthetic construct
  source 1..20: mol_type = other RNA
gggctcatggacccctgcac

SEQ ID NO: 20058 - RNA, 20 nt, synthetic construct
  source 1..20: mol_type = other RNA
aggggtccatgagcccccaa

SEQ ID NO: 20059 - RNA, 20 nt, synthetic construct
  source 1..20: mol_type = other RNA
actgcacctttgggggctca

SEQ ID NO: 20060 - RNA, 20 nt, synthetic construct
  source 1..20: mol_type = other RNA
ccaaaggtgcagtgagttgt

SEQ ID NO: 20061 - RNA, 20 nt, synthetic construct
  source 1..20: mol_type = other RNA
acaactcactgcacctttgg

SEQ ID NO: 20062 - RNA, 20 nt, synthetic construct
  source 1..20: mol_type = other RNA
tacaactcactgcacctttg

SEQ ID NO: 20063 - RNA, 20 nt, synthetic construct
  source 1..20: mol_type = other RNA
ctacaactcactgcaccttt

SEQ ID NO: 20064 - RNA, 20 nt, synthetic construct
  source 1..20: mol_type = other RNA
cctacaactcactgcacctt

SEQ ID NO: 20065 - RNA, 20 nt, synthetic construct
  source 1..20: mol_type = other RNA
tttctgaagaaagagtttgt

SEQ ID NO: 20066 - RNA, 20 nt, synthetic construct
  source 1..20: mol_type = other RNA
ggtttcatcagatcatcaga

SEQ ID NO: 20067 - RNA, 20 nt, synthetic construct
  source 1..20: mol_type = other RNA
tcatcagatcatcagaaggc

SEQ ID NO: 20068 - RNA, 20 nt, synthetic construct
  source 1..20: mol_type = other RNA
catcagatcatcagaaggct

SEQ ID NO: 20069 - RNA, 20 nt, synthetic construct
  source 1..20: mol_type = other RNA
cagaaggctgggtgtccctg

SEQ ID NO: 20070 - RNA, 20 nt, synthetic construct
  source 1..20: mol_type = other RNA
gtgtccctgtggagtgctga

SEQ ID NO: 20071 - RNA, 20 nt, synthetic construct
  source 1..20: mol_type = other RNA
tgtccctgtggagtgctgac

SEQ ID NO: 20072 - RNA, 20 nt, synthetic construct
  source 1..20: mol_type = other RNA
gtccctgtggagtgctgacg

SEQ ID NO: 20073 - RNA, 20 nt, synthetic construct
  source 1..20: mol_type = other RNA
ggccccgtcagcactccaca

SEQ ID NO: 20074 - RNA, 20 nt, synthetic construct
  source 1..20: mol_type = other RNA
cggccccgtcagcactccac

SEQ ID NO: 20075 - RNA, 20 nt, synthetic construct
  source 1..20: mol_type = other RNA
tgacggggccgtgtgcactg

SEQ ID NO: 20076 - RNA, 20 nt, synthetic construct
  source 1..20: mol_type = other RNA
gacggggccgtgtgcactgc

SEQ ID NO: 20077 - RNA, 20 nt, synthetic construct
  source 1..20: mol_type = other RNA
aacgtggagcaaaaagcact

SEQ ID NO: 20078 - RNA, 20 nt, synthetic construct
  source 1..20: mol_type = other RNA
aaacgtggagcaaaaagcac

SEQ ID NO: 20079 - RNA, 20 nt, synthetic construct
  source 1..20: mol_type = other RNA
acagctagagaacagaaacg

SEQ ID NO: 20080 - RNA, 20 nt, synthetic construct
  source 1..20: mol_type = other RNA
gtctgtgtcctagagaaagc

SEQ ID NO: 20081 - RNA, 20 nt, synthetic construct
  source 1..20: mol_type = other RNA
tctgtgtcctagagaaagcc

SEQ ID NO: 20082 - RNA, 20 nt, synthetic construct
  source 1..20: mol_type = other RNA
aagtgggcccggctttctct

SEQ ID NO: 20083 - RNA, 20 nt, synthetic construct
  source 1..20: mol_type = other RNA
gaggtgggggcaagtgggcc

SEQ ID NO: 20084 - RNA, 20 nt, synthetic construct
  source 1..20: mol_type = other RNA
ggggagaggtgggggcaagt

SEQ ID NO: 20085 - RNA, 20 nt, synthetic construct
  source 1..20: mol_type = other RNA
tggggagaggtgggggcaag

SEQ ID NO: 20086 - RNA, 20 nt, synthetic construct
  source 1..20: mol_type = other RNA
cagaaggtggggagaggtgg

SEQ ID NO: 20087 - RNA, 20 nt, synthetic construct
  source 1..20: mol_type = other RNA
gcagaaggtggggagaggtg

SEQ ID NO: 20088 - RNA, 20 nt, synthetic construct
  source 1..20: mol_type = other RNA
ggcagaaggtggggagaggt

SEQ ID NO: 20089 - RNA, 20 nt, synthetic construct
  source 1..20: mol_type = other RNA
gggcagaaggtggggagagg

SEQ ID NO: 20090 - RNA, 20 nt, synthetic construct
  source 1..20: mol_type = other RNA
agggggcagaaggtggggag

SEQ ID NO: 20091 - RNA, 20 nt, synthetic construct
  source 1..20: mol_type = other RNA
gggggagggggcagaaggtg

SEQ ID NO: 20092 - RNA, 20 nt, synthetic construct
  source 1..20: mol_type = other RNA
agggggagggggcagaaggt

SEQ ID NO: 20093 - RNA, 20 nt, synthetic construct
  source 1..20: mol_type = other RNA
cagggggagggggcagaagg

SEQ ID NO: 20094 - RNA, 20 nt, synthetic construct
  source 1..20: mol_type = other RNA
tggcagggggagggggcaga

SEQ ID NO: 20095 - RNA, 20 nt, synthetic construct
  source 1..20: mol_type = other RNA
gcgcagctggcagggggagg

SEQ ID NO: 20096 - RNA, 20 nt, synthetic construct
  source 1..20: mol_type = other RNA
ggcgcagctggcagggggag

SEQ ID NO: 20097 - RNA, 20 nt, synthetic construct
  source 1..20: mol_type = other RNA
aggcgcagctggcaggggga

SEQ ID NO: 20098 - RNA, 20 nt, synthetic construct
  source 1..20: mol_type = other RNA
gaggcgcagctggcaggggg

SEQ ID NO: 20099 - RNA, 20 nt, synthetic construct
  source 1..20: mol_type = other RNA
atggaggcgcagctggcagg

SEQ ID NO: 20100 - RNA, 20 nt, synthetic construct
  source 1..20: mol_type = other RNA
catggaggcgcagctggcag

SEQ ID NO: 20101 - RNA, 20 nt, synthetic construct
  source 1..20: mol_type = other RNA
acatggaggcgcagctggca

SEQ ID NO: 20102 - RNA, 20 nt, synthetic construct
  source 1..20: mol_type = other RNA
tacatggaggcgcagctggc

SEQ ID NO: 20103 - RNA, 20 nt, synthetic construct
  source 1..20: mol_type = other RNA
tacttacatggaggcgcagc

SEQ ID NO: 20104 - RNA, 20 nt, synthetic construct
  source 1..20: mol_type = other RNA
gactcaaagtacttacatgg

SEQ ID NO: 20105 - RNA, 20 nt, synthetic construct
  source 1..20: mol_type = other RNA
agggactcaaagtacttaca

SEQ ID NO: 20106 - RNA, 20 nt, synthetic construct
  source 1..20: mol_type = other RNA
ttgagtcccttaacacccca

SEQ ID NO: 20107 - RNA, 20 nt, synthetic construct
  source 1..20: mol_type = other RNA
cttaacaccccaaggcgtgt

SEQ ID NO: 20108 - RNA, 20 nt, synthetic construct
  source 1..20: mol_type = other RNA
aacacgccttggggtgttaa

SEQ ID NO: 20109 - RNA, 20 nt, synthetic construct
  source 1..20: mol_type = other RNA
caacacgccttggggtgtta

SEQ ID NO: 20110 - RNA, 20 nt, synthetic construct
  source 1..20: mol_type = other RNA
ctggccaccaacacgccttg

SEQ ID NO: 20111 - RNA, 20 nt, synthetic construct
  source 1..20: mol_type = other RNA
gctggccaccaacacgcctt

SEQ ID NO: 20112 - RNA, 20 nt, synthetic construct
  source 1..20: mol_type = other RNA
agctggccaccaacacgcct

SEQ ID NO: 20113 - RNA, 20 nt, synthetic construct
  source 1..20: mol_type = other RNA
cttgtcatcacgacaaaagc

SEQ ID NO: 20114 - RNA, 20 nt, synthetic construct
  source 1..20: mol_type = other RNA
acaagccccagcaagtctac

SEQ ID NO: 20115 - RNA, 20 nt, synthetic construct
  source 1..20: mol_type = other RNA
caagccccagcaagtctaca

SEQ ID NO: 20116 - RNA, 20 nt, synthetic construct
  source 1..20: mol_type = other RNA
cccagcaagtctacagggac

SEQ ID NO: 20117 - RNA, 20 nt, synthetic construct
  source 1..20: mol_type = other RNA
cagtccctgtagacttgctg

SEQ ID NO: 20118 - RNA, 20 nt, synthetic construct
  source 1..20: mol_type = other RNA
ccagtccctgtagacttgct

SEQ ID NO: 20119 - RNA, 20 nt, synthetic construct
  source 1..20: mol_type = other RNA
gccagtccctgtagacttgc

SEQ ID NO: 20120 - RNA, 20 nt, synthetic construct
  source 1..20: mol_type = other RNA
agggactggctgctttcatg

SEQ ID NO: 20121 - RNA, 20 nt, synthetic construct
  source 1..20: mol_type = other RNA
gggactggctgctttcatgt

SEQ ID NO: 20122 - RNA, 20 nt, synthetic construct
  source 1..20: mol_type = other RNA
gctgctttcatgtgggccct

SEQ ID NO: 20123 - RNA, 20 nt, synthetic construct
  source 1..20: mol_type = other RNA
ggccctcggtgaagcctcct

SEQ ID NO: 20124 - RNA, 20 nt, synthetic construct
  source 1..20: mol_type = other RNA
gaccaaggaggcttcaccga

SEQ ID NO: 20125 - RNA, 20 nt, synthetic construct
  source 1..20: mol_type = other RNA
agaccaaggaggcttcaccg

SEQ ID NO: 20126 - RNA, 20 nt, synthetic construct
  source 1..20: mol_type = other RNA
gaagcctccttggtctcagc

SEQ ID NO: 20127 - RNA, 20 nt, synthetic construct
  source 1..20: mol_type = other RNA
agggcctgctgagaccaagg

SEQ ID NO: 20128 - RNA, 20 nt, synthetic construct
  source 1..20: mol_type = other RNA
cacagggcctgctgagacca

SEQ ID NO: 20129 - RNA, 20 nt, synthetic construct
  source 1..20: mol_type = other RNA
ggccctgtgttgtacccacc

SEQ ID NO: 20130 - RNA, 20 nt, synthetic construct
  source 1..20: mol_type = other RNA
ggcctggtgggtacaacaca

SEQ ID NO: 20131 - RNA, 20 nt, synthetic construct
  source 1..20: mol_type = other RNA
gttgtacccaccaggcctct

SEQ ID NO: 20132 - RNA, 20 nt, synthetic construct
  source 1..20: mol_type = other RNA
caccaggcctctaggagatt

SEQ ID NO: 20133 - RNA, 20 nt, synthetic construct
  source 1..20: mol_type = other RNA
accaggcctctaggagatta

SEQ ID NO: 20134 - RNA, 20 nt, synthetic construct
  source 1..20: mol_type = other RNA
ccaggcctctaggagattag

SEQ ID NO: 20135 - RNA, 20 nt, synthetic construct
  source 1..20: mol_type = other RNA
taatctcctagaggcctggt

SEQ ID NO: 20136 - RNA, 20 nt, synthetic construct
  source 1..20: mol_type = other RNA
ctaatctcctagaggcctgg

SEQ ID NO: 20137 - RNA, 20 nt, synthetic construct
  source 1..20: mol_type = other RNA
cccctaatctcctagaggcc

SEQ ID NO: 20138 - RNA, 20 nt, synthetic construct
  source 1..20: mol_type = other RNA
gaagccccctaatctcctag

SEQ ID NO: 20139 - RNA, 20 nt, synthetic construct
  source 1..20: mol_type = other RNA
ggggcttctgtggctccaga

SEQ ID NO: 20140 - RNA, 20 nt, synthetic construct
  source 1..20: mol_type = other RNA
gggaaaagctttgagccatc

SEQ ID NO: 20141 - RNA, 20 nt, synthetic construct
  source 1..20: mol_type = other RNA
ctagggataacacagaggaa

SEQ ID NO: 20142 - RNA, 20 nt, synthetic construct
  source 1..20: mol_type = other RNA
gctagggataacacagagga

SEQ ID NO: 20143 - RNA, 20 nt, synthetic construct
  source 1..20: mol_type = other RNA
tgtgttatccctagcccacc

SEQ ID NO: 20144 - RNA, 20 nt, synthetic construct
  source 1..20: mol_type = other RNA
gtgggctagggataacacag

SEQ ID NO: 20145 - RNA, 20 nt, synthetic construct
  source 1..20: mol_type = other RNA
gacggaagccaggtgggcta

SEQ ID NO: 20146 - RNA, 20 nt, synthetic construct
  source 1..20: mol_type = other RNA
ggacggaagccaggtgggct

SEQ ID NO: 20147 - RNA, 20 nt, synthetic construct
  source 1..20: mol_type = other RNA
cacctggcttccgtcctcac

SEQ ID NO: 20148 - RNA, 20 nt, synthetic construct
  source 1..20: mol_type = other RNA
agtgaggacggaagccaggt

SEQ ID NO: 20149 - RNA, 20 nt, synthetic construct
  source 1..20: mol_type = other RNA
cagtgaggacggaagccagg

SEQ ID NO: 20150 - RNA, 20 nt, synthetic construct
  source 1..20: mol_type = other RNA
gcttccgtcctcactggcca

SEQ ID NO: 20151 - RNA, 20 nt, synthetic construct
  source 1..20: mol_type = other RNA
cttccgtcctcactggccac

SEQ ID NO: 20152 - RNA, 20 nt, synthetic construct
  source 1..20: mol_type = other RNA
ttccgtcctcactggccacg

SEQ ID NO: 20153 - RNA, 20 nt, synthetic construct
  source 1..20: mol_type = other RNA
tcctcactggccacggggct

SEQ ID NO: 20154 - RNA, 20 nt, synthetic construct
  source 1..20: mol_type = other RNA
cctcactggccacggggctt

SEQ ID NO: 20155 - RNA, 20 nt, synthetic construct
  source 1..20: mol_type = other RNA
ctcactggccacggggcttg

SEQ ID NO: 20156 - RNA, 20 nt, synthetic construct
  source 1..20: mol_type = other RNA
tcactggccacggggcttgg

SEQ ID NO: 20157 - RNA, 20 nt, synthetic construct
  source 1..20: mol_type = other RNA
cccaagccccgtggccagtg

SEQ ID NO: 20158 - RNA, 20 nt, synthetic construct
  source 1..20: mol_type = other RNA
tgaaaatcccccaagccccg

SEQ ID NO: 20159 - RNA, 20 nt, synthetic construct
  source 1..20: mol_type = other RNA
ggggattttcagtctctcca

SEQ ID NO: 20160 - RNA, 20 nt, synthetic construct
  source 1..20: mol_type = other RNA
tttcagtctctccaaggctc

SEQ ID NO: 20161 - RNA, 20 nt, synthetic construct
  source 1..20: mol_type = other RNA
ggctctggcatcttccagag

SEQ ID NO: 20162 - RNA, 20 nt, synthetic construct
  source 1..20: mol_type = other RNA
gctctggcatcttccagagt

SEQ ID NO: 20163 - RNA, 20 nt, synthetic construct
  source 1..20: mol_type = other RNA
cttccagagtgggctagtct

SEQ ID NO: 20164 - RNA, 20 nt, synthetic construct
  source 1..20: mol_type = other RNA
actccaagactagcccactc

SEQ ID NO: 20165 - RNA, 20 nt, synthetic construct
  source 1..20: mol_type = other RNA
gacagaaagaatggctcaga

SEQ ID NO: 20166 - RNA, 20 nt, synthetic construct
  source 1..20: mol_type = other RNA
attctttctgtcaccactgc

SEQ ID NO: 20167 - RNA, 20 nt, synthetic construct
  source 1..20: mol_type = other RNA
ttctttctgtcaccactgct

SEQ ID NO: 20168 - RNA, 20 nt, synthetic construct
  source 1..20: mol_type = other RNA
agcagtggtgacagaaagaa

SEQ ID NO: 20169 - RNA, 20 nt, synthetic construct
  source 1..20: mol_type = other RNA
ccactgctgggcctgcctgc

SEQ ID NO: 20170 - RNA, 20 nt, synthetic construct
  source 1..20: mol_type = other RNA
cactgctgggcctgcctgct

SEQ ID NO: 20171 - RNA, 20 nt, synthetic construct
  source 1..20: mol_type = other RNA
ccagcaggcaggcccagcag

SEQ ID NO: 20172 - RNA, 20 nt, synthetic construct
  source 1..20: mol_type = other RNA
gggcctgcctgctgggcctt

SEQ ID NO: 20173 - RNA, 20 nt, synthetic construct
  source 1..20: mol_type = other RNA
tcacctaaggcccagcaggc

SEQ ID NO: 20174 - RNA, 20 nt, synthetic construct
  source 1..20: mol_type = other RNA
gaagtcacctaaggcccagc

SEQ ID NO: 20175 - RNA, 20 nt, synthetic construct
  source 1..20: mol_type = other RNA
gccttaggtgacttcttgag

SEQ ID NO: 20176 - RNA, 20 nt, synthetic construct
  source 1..20: mol_type = other RNA
ttaggtgacttcttgagagg

SEQ ID NO: 20177 - RNA, 20 nt, synthetic construct
  source 1..20: mol_type = other RNA
acctctcaagaagtcaccta

SEQ ID NO: 20178 - RNA, 20 nt, synthetic construct
  source 1..20: mol_type = other RNA
tggccaaagctgctaatccc

SEQ ID NO: 20179 - RNA, 20 nt, synthetic construct
  source 1..20: mol_type = other RNA
caaagctgctaatccctgga

SEQ ID NO: 20180 - RNA, 20 nt, synthetic construct
  source 1..20: mol_type = other RNA
aaagctgctaatccctggaa

SEQ ID NO: 20181 - RNA, 20 nt, synthetic construct
  source 1..20: mol_type = other RNA
aagctgctaatccctggaag

SEQ ID NO: 20182 - RNA, 20 nt, synthetic construct
  source 1..20: mol_type = other RNA
cttccagggattagcagctt

SEQ ID NO: 20183 - RNA, 20 nt, synthetic construct
  source 1..20: mol_type = other RNA
aatccctggaaggggctcct

SEQ ID NO: 20184 - RNA, 20 nt, synthetic construct
  source 1..20: mol_type = other RNA
aatcctaggagccccttcca

SEQ ID NO: 20185 - RNA, 20 nt, synthetic construct
  source 1..20: mol_type = other RNA
aaatcctaggagccccttcc

SEQ ID NO: 20186 - RNA, 20 nt, synthetic construct
  source 1..20: mol_type = other RNA
gggctcctaggatttccctg

SEQ ID NO: 20187 - RNA, 20 nt, synthetic construct
  source 1..20: mol_type = other RNA
tcctaggatttccctgtggc

SEQ ID NO: 20188 - RNA, 20 nt, synthetic construct
  source 1..20: mol_type = other RNA
aggatttccctgtggctggc

SEQ ID NO: 20189 - RNA, 20 nt, synthetic construct
  source 1..20: mol_type = other RNA
gccagccacagggaaatcct

SEQ ID NO: 20190 - RNA, 20 nt, synthetic construct
  source 1..20: mol_type = other RNA
cctgtggctggcaggaccct

SEQ ID NO: 20191 - RNA, 20 nt, synthetic construct
  source 1..20: mol_type = other RNA
caagggtcctgccagccaca

SEQ ID NO: 20192 - RNA, 20 nt, synthetic construct
  source 1..20: mol_type = other RNA
ccaagggtcctgccagccac

SEQ ID NO: 20193 - RNA, 20 nt, synthetic construct
  source 1..20: mol_type = other RNA
aggacccttggccacccacg

SEQ ID NO: 20194 - RNA, 20 nt, synthetic construct
  source 1..20: mol_type = other RNA
cacaccacgtgggtggccaa

SEQ ID NO: 20195 - RNA, 20 nt, synthetic construct
  source 1..20: mol_type = other RNA
tcacaccacgtgggtggcca

SEQ ID NO: 20196 - RNA, 20 nt, synthetic construct
  source 1..20: mol_type = other RNA
cacccacgtggtgtgacatg

SEQ ID NO: 20197 - RNA, 20 nt, synthetic construct
  source 1..20: mol_type = other RNA
ctcatgtcacaccacgtggg

SEQ ID NO: 20198 - RNA, 20 nt, synthetic construct
  source 1..20: mol_type = other RNA
gtggtgtgacatgaggagcc

SEQ ID NO: 20199 - RNA, 20 nt, synthetic construct
  source 1..20: mol_type = other RNA
gctcctcatgtcacaccacg

SEQ ID NO: 20200 - RNA, 20 nt, synthetic construct
  source 1..20: mol_type = other RNA
ggaggttgggctggctttcc

SEQ ID NO: 20201 - RNA, 20 nt, synthetic construct
  source 1..20: mol_type = other RNA
cttaaggatggaggttgggc

SEQ ID NO: 20202 - RNA, 20 nt, synthetic construct
  source 1..20: mol_type = other RNA
ggggcttaaggatggaggtt

SEQ ID NO: 20203 - RNA, 20 nt, synthetic construct
  source 1..20: mol_type = other RNA
tggggcttaaggatggaggt

SEQ ID NO: 20204 - RNA, 20 nt, synthetic construct
  source 1..20: mol_type = other RNA
tacgtggggcttaaggatgg

SEQ ID NO: 20205 - RNA, 20 nt, synthetic construct
  source 1..20: mol_type = other RNA
ttatacgtggggcttaagga

SEQ ID NO: 20206 - RNA, 20 nt, synthetic construct
  source 1..20: mol_type = other RNA
atgtttatacgtggggctta

SEQ ID NO: 20207 - RNA, 20 nt, synthetic construct
  source 1..20: mol_type = other RNA
aaaaggtatgtttatacgtg

SEQ ID NO: 20208 - RNA, 20 nt, synthetic construct
  source 1..20: mol_type = other RNA
aaaaaggtatgtttatacgt

SEQ ID NO: 20209 - RNA, 20 nt, synthetic construct
  source 1..20: mol_type = other RNA
aaaaaaggtatgtttatacg

SEQ ID NO: 20210 - RNA, 20 nt, synthetic construct
  source 1..20: mol_type = other RNA
tgcagttaaaaaaaaaaaaa

SEQ ID NO: 20211 - RNA, 20 nt, synthetic construct
  source 1..20: mol_type = other RNA
cctgcagttctactgttgtc

SEQ ID NO: 20212 - RNA, 20 nt, synthetic construct
  source 1..20: mol_type = other RNA
cctgacaacagtagaactgc

SEQ ID NO: 20213 - RNA, 20 nt, synthetic construct
  source 1..20: mol_type = other RNA
aggttgccttgtgctctcct

SEQ ID NO: 20214 - RNA, 20 nt, synthetic construct
  source 1..20: mol_type = other RNA
aggatgccaaggagagcaca

SEQ ID NO: 20215 - RNA, 20 nt, synthetic construct
  source 1..20: mol_type = other RNA
ctccttggcatcctctaaga

SEQ ID NO: 20216 - RNA, 20 nt, synthetic construct
  source 1..20: mol_type = other RNA
tgccttcttagaggatgcca

SEQ ID NO: 20217 - RNA, 20 nt, synthetic construct
  source 1..20: mol_type = other RNA
aaaggtatttgccttcttag

SEQ ID NO: 20218 - RNA, 20 nt, synthetic construct
  source 1..20: mol_type = other RNA
aaggcaaataccttttcagc

SEQ ID NO: 20219 - RNA, 20 nt, synthetic construct
  source 1..20: mol_type = other RNA
aggcaaataccttttcagct

SEQ ID NO: 20220 - RNA, 20 nt, synthetic construct
  source 1..20: mol_type = other RNA
ttaaaagcacccagctgaaa

SEQ ID NO: 20221 - RNA, 20 nt, synthetic construct
  source 1..20: mol_type = other RNA
tgctgtcaagaagcaagccc

SEQ ID NO: 20222 - RNA, 20 nt, synthetic construct
  source 1..20: mol_type = other RNA
gaagcaagccctggccagcc

SEQ ID NO: 20223 - RNA, 20 nt, synthetic construct
  source 1..20: mol_type = other RNA
gaaaagggccaggctggcca

SEQ ID NO: 20224 - RNA, 20 nt, synthetic construct
  source 1..20: mol_type = other RNA
ggaaaagggccaggctggcc

SEQ ID NO: 20225 - RNA, 20 nt, synthetic construct
  source 1..20: mol_type = other RNA
acactggaaaagggccaggc

SEQ ID NO: 20226 - RNA, 20 nt, synthetic construct
  source 1..20: mol_type = other RNA
cagaacactggaaaagggcc

SEQ ID NO: 20227 - RNA, 20 nt, synthetic construct
  source 1..20: mol_type = other RNA
tcacacagaacactggaaaa

SEQ ID NO: 20228 - RNA, 20 nt, synthetic construct
  source 1..20: mol_type = other RNA
gtcacacagaacactggaaa

SEQ ID NO: 20229 - RNA, 20 nt, synthetic construct
  source 1..20: mol_type = other RNA
gccacggtcacacagaacac

SEQ ID NO: 20230 - RNA, 20 nt, synthetic construct
  source 1..20: mol_type = other RNA
gaagagaagcaacttggcca

SEQ ID NO: 20231 - RNA, 20 nt, synthetic construct
  source 1..20: mol_type = other RNA
ccaagttgcttctcttctct

SEQ ID NO: 20232 - RNA, 20 nt, synthetic construct
  source 1..20: mol_type = other RNA
cccagagaagagaagcaact

SEQ ID NO: 20233 - RNA, 20 nt, synthetic construct
  source 1..20: mol_type = other RNA
ttttcagctctagcactttg

SEQ ID NO: 20234 - RNA, 20 nt, synthetic construct
  source 1..20: mol_type = other RNA
caaagtgctagagctgaaaa

SEQ ID NO: 20235 - RNA, 20 nt, synthetic construct
  source 1..20: mol_type = other RNA
tcaaagtgctagagctgaaa

SEQ ID NO: 20236 - RNA, 20 nt, synthetic construct
  source 1..20: mol_type = other RNA
agcactttgaggctccagca

SEQ ID NO: 20237 - RNA, 20 nt, synthetic construct
  source 1..20: mol_type = other RNA
gagggtgtaagaatccatgc

SEQ ID NO: 20238 - RNA, 20 nt, synthetic construct
  source 1..20: mol_type = other RNA
tacaccctccacacctttgc

SEQ ID NO: 20239 - RNA, 20 nt, synthetic construct
  source 1..20: mol_type = other RNA
gtgaccggcaaaggtgtgga

SEQ ID NO: 20240 - RNA, 20 nt, synthetic construct
  source 1..20: mol_type = other RNA
ggtgaccggcaaaggtgtgg

SEQ ID NO: 20241 - RNA, 20 nt, synthetic construct
  source 1..20: mol_type = other RNA
aaaggtgaccggcaaaggtg

SEQ ID NO: 20242 - RNA, 20 nt, synthetic construct
  source 1..20: mol_type = other RNA
ggaagaaaggtgaccggcaa

SEQ ID NO: 20243 - RNA, 20 nt, synthetic construct
  source 1..20: mol_type = other RNA
agagaaggaagaaaggtgac

SEQ ID NO: 20244 - RNA, 20 nt, synthetic construct
  source 1..20: mol_type = other RNA
acctttcttccttctctgca

SEQ ID NO: 20245 - RNA, 20 nt, synthetic construct
  source 1..20: mol_type = other RNA
tttcttccttctctgcaggg

SEQ ID NO: 20246 - RNA, 20 nt, synthetic construct
  source 1..20: mol_type = other RNA
ttcttccttctctgcagggt

SEQ ID NO: 20247 - RNA, 20 nt, synthetic construct
  source 1..20: mol_type = other RNA
tcttccttctctgcagggtg

SEQ ID NO: 20248 - RNA, 20 nt, synthetic construct
  source 1..20: mol_type = other RNA
accctgcagagaaggaagaa

SEQ ID NO: 20249 - RNA, 20 nt, synthetic construct
  source 1..20: mol_type = other RNA
ttctctgcagggtggggcac

SEQ ID NO: 20250 - RNA, 20 nt, synthetic construct
  source 1..20: mol_type = other RNA
tctctgcagggtggggcaca

SEQ ID NO: 20251 - RNA, 20 nt, synthetic construct
  source 1..20: mol_type = other RNA
tgtgccccaccctgcagaga

SEQ ID NO: 20252 - RNA, 20 nt, synthetic construct
  source 1..20: mol_type = other RNA
tgcagggtggggcacaggga

SEQ ID NO: 20253 - RNA, 20 nt, synthetic construct
  source 1..20: mol_type = other RNA
gcagggtggggcacagggaa

SEQ ID NO: 20254 - RNA, 20 nt, synthetic construct
  source 1..20: mol_type = other RNA
gtggggcacagggaagggcc

SEQ ID NO: 20255 - RNA, 20 nt, synthetic construct
  source 1..20: mol_type = other RNA
gaagggcctggcagctgagc

SEQ ID NO: 20256 - RNA, 20 nt, synthetic construct
  source 1..20: mol_type = other RNA
aagggcctggcagctgagct

SEQ ID NO: 20257 - RNA, 20 nt, synthetic construct
  source 1..20: mol_type = other RNA
ggcctggcagctgagctggg

SEQ ID NO: 20258 - RNA, 20 nt, synthetic construct
  source 1..20: mol_type = other RNA
gcctggcagctgagctgggt

SEQ ID NO: 20259 - RNA, 20 nt, synthetic construct
  source 1..20: mol_type = other RNA
cctggcagctgagctgggtg

SEQ ID NO: 20260 - RNA, 20 nt, synthetic construct
  source 1..20: mol_type = other RNA
cagctgagctgggtggggcc

SEQ ID NO: 20261 - RNA, 20 nt, synthetic construct
  source 1..20: mol_type = other RNA
agctgagctgggtggggcca

SEQ ID NO: 20262 - RNA, 20 nt, synthetic construct
  source 1..20: mol_type = other RNA
gctgagctgggtggggccag

SEQ ID NO: 20263 - RNA, 20 nt, synthetic construct
  source 1..20: mol_type = other RNA
tgatgctggcttttggcccc

SEQ ID NO: 20264 - RNA, 20 nt, synthetic construct
  source 1..20: mol_type = other RNA
gtgtctatgatgctggcttt

SEQ ID NO: 20265 - RNA, 20 nt, synthetic construct
  source 1..20: mol_type = other RNA
gggaaaagtgtctatgatgc

SEQ ID NO: 20266 - RNA, 20 nt, synthetic construct
  source 1..20: mol_type = other RNA
tagacacttttccctccagc

SEQ ID NO: 20267 - RNA, 20 nt, synthetic construct
  source 1..20: mol_type = other RNA
agacacttttccctccagct

SEQ ID NO: 20268 - RNA, 20 nt, synthetic construct
  source 1..20: mol_type = other RNA
gactggtatgcccagctgga

SEQ ID NO: 20269 - RNA, 20 nt, synthetic construct
  source 1..20: mol_type = other RNA
ggactggtatgcccagctgg

SEQ ID NO: 20270 - RNA, 20 nt, synthetic construct
  source 1..20: mol_type = other RNA
gaaggactggtatgcccagc

SEQ ID NO: 20271 - RNA, 20 nt, synthetic construct
  source 1..20: mol_type = other RNA
cagtccttcctcttcttctc

SEQ ID NO: 20272 - RNA, 20 nt, synthetic construct
  source 1..20: mol_type = other RNA
ctgagaagaagaggaaggac

SEQ ID NO: 20273 - RNA, 20 nt, synthetic construct
  source 1..20: mol_type = other RNA
cttcctcttcttctcaggac

SEQ ID NO: 20274 - RNA, 20 nt, synthetic construct
  source 1..20: mol_type = other RNA
cctcttcttctcaggacagg

SEQ ID NO: 20275 - RNA, 20 nt, synthetic construct
  source 1..20: mol_type = other RNA
ctgtcctgagaagaagagga

SEQ ID NO: 20276 - RNA, 20 nt, synthetic construct
  source 1..20: mol_type = other RNA
tcttcttctcaggacaggtg

SEQ ID NO: 20277 - RNA, 20 nt, synthetic construct
  source 1..20: mol_type = other RNA
ccacctgtcctgagaagaag

SEQ ID NO: 20278 - RNA, 20 nt, synthetic construct
  source 1..20: mol_type = other RNA
caggacaggtggggaaactg

SEQ ID NO: 20279 - RNA, 20 nt, synthetic construct
  source 1..20: mol_type = other RNA
caggtggggaaactgaggtc

SEQ ID NO: 20280 - RNA, 20 nt, synthetic construct
  source 1..20: mol_type = other RNA
gtggggaaactgaggtctgg

SEQ ID NO: 20281 - RNA, 20 nt, synthetic construct
  source 1..20: mol_type = other RNA
tggggaaactgaggtctgga

SEQ ID NO: 20282 - RNA, 20 nt, synthetic construct
  source 1..20: mol_type = other RNA
ggggaaactgaggtctggag

SEQ ID NO: 20283 - RNA, 20 nt, synthetic construct
  source 1..20: mol_type = other RNA
gggaaactgaggtctggagg

SEQ ID NO: 20284 - RNA, 20 nt, synthetic construct
  source 1..20: mol_type = other RNA
aactgaggtctggaggggga

SEQ ID NO: 20285 - RNA, 20 nt, synthetic construct
  source 1..20: mol_type = other RNA
actgaggtctggagggggaa

SEQ ID NO: 20286 - RNA, 20 nt, synthetic construct
  source 1..20: mol_type = other RNA
ggtctggagggggaagggcc

SEQ ID NO: 20287 - RNA, 20 nt, synthetic construct
  source 1..20: mol_type = other RNA
gtctggagggggaagggcca

SEQ ID NO: 20288 - RNA, 20 nt, synthetic construct
  source 1..20: mol_type = other RNA
ggagggggaagggccagggc

SEQ ID NO: 20289 - RNA, 20 nt, synthetic construct
  source 1..20: mol_type = other RNA
gaagggccagggctggaacc

SEQ ID NO: 20290 - RNA, 20 nt, synthetic construct
  source 1..20: mol_type = other RNA
ctgggtcctggttccagccc

SEQ ID NO: 20291 - RNA, 20 nt, synthetic construct
  source 1..20: mol_type = other RNA
caataaggataactgggtcc

SEQ ID NO: 20292 - RNA, 20 nt, synthetic construct
  source 1..20: mol_type = other RNA
cactggcaataaggataact

SEQ ID NO: 20293 - RNA, 20 nt, synthetic construct
  source 1..20: mol_type = other RNA
tcactggcaataaggataac

SEQ ID NO: 20294 - RNA, 20 nt, synthetic construct
  source 1..20: mol_type = other RNA
aggagcactcactggcaata

SEQ ID NO: 20295 - RNA, 20 nt, synthetic construct
  source 1..20: mol_type = other RNA
gtgagtgctcctcctgctgt

SEQ ID NO: 20296 - RNA, 20 nt, synthetic construct
  source 1..20: mol_type = other RNA
acagcaggaggagcactcac

SEQ ID NO: 20297 - RNA, 20 nt, synthetic construct
  source 1..20: mol_type = other RNA
aggtagcagccaacagcagg

SEQ ID NO: 20298 - RNA, 20 nt, synthetic construct
  source 1..20: mol_type = other RNA
gagaggtagcagccaacagc

SEQ ID NO: 20299 - RNA, 20 nt, synthetic construct
  source 1..20: mol_type = other RNA
tggctgctacctctcttgag

SEQ ID NO: 20300 - RNA, 20 nt, synthetic construct
  source 1..20: mol_type = other RNA
ggctgctacctctcttgaga

SEQ ID NO: 20301 - RNA, 20 nt, synthetic construct
  source 1..20: mol_type = other RNA
tcttctgaccctctcaagag

SEQ ID NO: 20302 - RNA, 20 nt, synthetic construct
  source 1..20: mol_type = other RNA
tcagaagacccactagcatg

SEQ ID NO: 20303 - RNA, 20 nt, synthetic construct
  source 1..20: mol_type = other RNA
cagaagacccactagcatga

SEQ ID NO: 20304 - RNA, 20 nt, synthetic construct
  source 1..20: mol_type = other RNA
gacccactagcatgagggtc

SEQ ID NO: 20305 - RNA, 20 nt, synthetic construct
  source 1..20: mol_type = other RNA
acccactagcatgagggtca

SEQ ID NO: 20306 - RNA, 20 nt, synthetic construct
  source 1..20: mol_type = other RNA
tccctgaccctcatgctagt

SEQ ID NO: 20307 - RNA, 20 nt, synthetic construct
  source 1..20: mol_type = other RNA
gtccctgaccctcatgctag

SEQ ID NO: 20308 - RNA, 20 nt, synthetic construct
  source 1..20: mol_type = other RNA
acatgctttttcctttcccg

SEQ ID NO: 20309 - RNA, 20 nt, synthetic construct
  source 1..20: mol_type = other RNA
gctttttcctttcccgtgga

SEQ ID NO: 20310 - RNA, 20 nt, synthetic construct
  source 1..20: mol_type = other RNA
ttcccgtggaaggctcctcc

SEQ ID NO: 20311 - RNA, 20 nt, synthetic construct
  source 1..20: mol_type = other RNA
ggaggagccttccacgggaa

SEQ ID NO: 20312 - RNA, 20 nt, synthetic construct
  source 1..20: mol_type = other RNA
cgtggaaggctcctccaggc

SEQ ID NO: 20313 - RNA, 20 nt, synthetic construct
  source 1..20: mol_type = other RNA
gtggaaggctcctccaggca

SEQ ID NO: 20314 - RNA, 20 nt, synthetic construct
  source 1..20: mol_type = other RNA
tgcctggaggagccttccac

SEQ ID NO: 20315 - RNA, 20 nt, synthetic construct
  source 1..20: mol_type = other RNA
ctgcctggaggagccttcca

SEQ ID NO: 20316 - RNA, 20 nt, synthetic construct
  source 1..20: mol_type = other RNA
aggctcctccaggcagggct

SEQ ID NO: 20317 - RNA, 20 nt, synthetic construct
  source 1..20: mol_type = other RNA
ggctcctccaggcagggctt

SEQ ID NO: 20318 - RNA, 20 nt, synthetic construct
  source 1..20: mol_type = other RNA
ctccaggcagggcttgggtg

SEQ ID NO: 20319 - RNA, 20 nt, synthetic construct
  source 1..20: mol_type = other RNA
ctcacccaagccctgcctgg

SEQ ID NO: 20320 - RNA, 20 nt, synthetic construct
  source 1..20: mol_type = other RNA
tgcctcacccaagccctgcc

SEQ ID NO: 20321 - RNA, 20 nt, synthetic construct
  source 1..20: mol_type = other RNA
gggcttgggtgaggcaggcg

SEQ ID NO: 20322 - RNA, 20 nt, synthetic construct
  source 1..20: mol_type = other RNA
tgaggcaggcgaggtgccag

SEQ ID NO: 20323 - RNA, 20 nt, synthetic construct
  source 1..20: mol_type = other RNA
gcgaggtgccagtggttccc

SEQ ID NO: 20324 - RNA, 20 nt, synthetic construct
  source 1..20: mol_type = other RNA
cgaggtgccagtggttccct

SEQ ID NO: 20325 - RNA, 20 nt, synthetic construct
  source 1..20: mol_type = other RNA
tgccagtggttccctgggca

SEQ ID NO: 20326 - RNA, 20 nt, synthetic construct
  source 1..20: mol_type = other RNA
gccagtggttccctgggcac

SEQ ID NO: 20327 - RNA, 20 nt, synthetic construct
  source 1..20: mol_type = other RNA
ccagtggttccctgggcacg

SEQ ID NO: 20328 - RNA, 20 nt, synthetic construct
  source 1..20: mol_type = other RNA
ccccgtgcccagggaaccac

SEQ ID NO: 20329 - RNA, 20 nt, synthetic construct
  source 1..20: mol_type = other RNA
ccctgggcacggggcagaat

SEQ ID NO: 20330 - RNA, 20 nt, synthetic construct
  source 1..20: mol_type = other RNA
tgggcacggggcagaatcgg

SEQ ID NO: 20331 - RNA, 20 nt, synthetic construct
  source 1..20: mol_type = other RNA
ccgattctgccccgtgccca

SEQ ID NO: 20332 - RNA, 20 nt, synthetic construct
  source 1..20: mol_type = other RNA
gcacggggcagaatcggagg

SEQ ID NO: 20333 - RNA, 20 nt, synthetic construct
  source 1..20: mol_type = other RNA
aggaggacatcctctttctg

SEQ ID NO: 20334 - RNA, 20 nt, synthetic construct
  source 1..20: mol_type = other RNA
acatcctctttctgaggtta

SEQ ID NO: 20335 - RNA, 20 nt, synthetic construct
  source 1..20: mol_type = other RNA
tcctctttctgaggttaagg

SEQ ID NO: 20336 - RNA, 20 nt, synthetic construct
  source 1..20: mol_type = other RNA
ctttctgaggttaaggaggt

SEQ ID NO: 20337 - RNA, 20 nt, synthetic construct
  source 1..20: mol_type = other RNA
tttctgaggttaaggaggta

SEQ ID NO: 20338 - RNA, 20 nt, synthetic construct
  source 1..20: mol_type = other RNA
ttctgaggttaaggaggtag

SEQ ID NO: 20339 - RNA, 20 nt, synthetic construct
  source 1..20: mol_type = other RNA
gaggttaaggaggtaggggc

SEQ ID NO: 20340 - RNA, 20 nt, synthetic construct
  source 1..20: mol_type = other RNA
gttaaggaggtaggggctgg

SEQ ID NO: 20341 - RNA, 20 nt, synthetic construct
  source 1..20: mol_type = other RNA
aggggctggaggccttgaca

SEQ ID NO: 20342 - RNA, 20 nt, synthetic construct
  source 1..20: mol_type = other RNA
ggggctggaggccttgacaa

SEQ ID NO: 20343 - RNA, 20 nt, synthetic construct
  source 1..20: mol_type = other RNA
gctggaggccttgacaaggg

SEQ ID NO: 20344 - RNA, 20 nt, synthetic construct
  source 1..20: mol_type = other RNA
ggaggccttgacaagggagg

SEQ ID NO: 20345 - RNA, 20 nt, synthetic construct
  source 1..20: mol_type = other RNA
tgacaagggaggtggcatga

SEQ ID NO: 20346 - RNA, 20 nt, synthetic construct
  source 1..20: mol_type = other RNA
gacaagggaggtggcatgaa

SEQ ID NO: 20347 - RNA, 20 nt, synthetic construct
  source 1..20: mol_type = other RNA
acaagggaggtggcatgaag

SEQ ID NO: 20348 - RNA, 20 nt, synthetic construct
  source 1..20: mol_type = other RNA
ggaggtggcatgaaggggcg

SEQ ID NO: 20349 - RNA, 20 nt, synthetic construct
  source 1..20: mol_type = other RNA
ggtggcatgaaggggcgtgg

SEQ ID NO: 20350 - RNA, 20 nt, synthetic construct
  source 1..20: mol_type = other RNA
gaaggggcgtggaggtttct

SEQ ID NO: 20351 - RNA, 20 nt, synthetic construct
  source 1..20: mol_type = other RNA
cgtggaggtttctaggaacg

SEQ ID NO: 20352 - RNA, 20 nt, synthetic construct
  source 1..20: mol_type = other RNA
gaggtttctaggaacgtggt

SEQ ID NO: 20353 - RNA, 20 nt, synthetic construct
  source 1..20: mol_type = other RNA
gtttctaggaacgtggttgg

SEQ ID NO: 20354 - RNA, 20 nt, synthetic construct
  source 1..20: mol_type = other RNA
aggaacgtggttggtggcgc

SEQ ID NO: 20355 - RNA, 20 nt, synthetic construct
  source 1..20: mol_type = other RNA
ggaacgtggttggtggcgca

SEQ ID NO: 20356 - RNA, 20 nt, synthetic construct
  source 1..20: mol_type = other RNA
ttggtggcgcagggtgctct

SEQ ID NO: 20357 - RNA, 20 nt, synthetic construct
  source 1..20: mol_type = other RNA
tggtggcgcagggtgctcta

SEQ ID NO: 20358 - RNA, 20 nt, synthetic construct
  source 1..20: mol_type = other RNA
gcagaagcaagggagggagg

SEQ ID NO: 20359 - RNA, 20 nt, synthetic construct
  source 1..20: mol_type = other RNA
aaggcagaagcaagggaggg

SEQ ID NO: 20360 - RNA, 20 nt, synthetic construct
  source 1..20: mol_type = other RNA
gggaaggcagaagcaaggga

SEQ ID NO: 20361 - RNA, 20 nt, synthetic construct
  source 1..20: mol_type = other RNA
agggaaggcagaagcaaggg

SEQ ID NO: 20362 - RNA, 20 nt, synthetic construct
  source 1..20: mol_type = other RNA
gaaagggaaggcagaagcaa

SEQ ID NO: 20363 - RNA, 20 nt, synthetic construct
  source 1..20: mol_type = other RNA
agaaagggaaggcagaagca

SEQ ID NO: 20364 - RNA, 20 nt, synthetic construct
  source 1..20: mol_type = other RNA
ttctgccttccctttctcct

SEQ ID NO: 20365 - RNA, 20 nt, synthetic construct
  source 1..20: mol_type = other RNA
tctgccttccctttctcctg

SEQ ID NO: 20366 - RNA, 20 nt, synthetic construct
  source 1..20: mol_type = other RNA
gccttccctttctcctgggg

SEQ ID NO: 20367 - RNA, 20 nt, synthetic construct
  source 1..20: mol_type = other RNA
ccttccctttctcctgggga

SEQ ID NO: 20368 - RNA, 20 nt, synthetic construct
  source 1..20: mol_type = other RNA
cttccctttctcctggggag

SEQ ID NO: 20369 - RNA, 20 nt, synthetic construct
  source 1..20: mol_type = other RNA
ccctccccaggagaaaggga

SEQ ID NO: 20370 - RNA, 20 nt, synthetic construct
  source 1..20: mol_type = other RNA
ctttctcctggggaggggac

SEQ ID NO: 20371 - RNA, 20 nt, synthetic construct
  source 1..20: mol_type = other RNA
tttctcctggggaggggact

SEQ ID NO: 20372 - RNA, 20 nt, synthetic construct
  source 1..20: mol_type = other RNA
agtcccctccccaggagaaa

SEQ ID NO: 20373 - RNA, 20 nt, synthetic construct
  source 1..20: mol_type = other RNA
cagtcccctccccaggagaa

SEQ ID NO: 20374 - RNA, 20 nt, synthetic construct
  source 1..20: mol_type = other RNA
gttggcccagtcccctcccc

SEQ ID NO: 20375 - RNA, 20 nt, synthetic construct
  source 1..20: mol_type = other RNA
aacagtaatgccatttttcc

SEQ ID NO: 20376 - RNA, 20 nt, synthetic construct
  source 1..20: mol_type = other RNA
aggaaaaatggcattactgt

SEQ ID NO: 20377 - RNA, 20 nt, synthetic construct
  source 1..20: mol_type = other RNA
aatgccatttttcctggccc

SEQ ID NO: 20378 - RNA, 20 nt, synthetic construct
  source 1..20: mol_type = other RNA
atgccatttttcctggccct

SEQ ID NO: 20379 - RNA, 20 nt, synthetic construct
  source 1..20: mol_type = other RNA
tttttcctggccctgggatt

SEQ ID NO: 20380 - RNA, 20 nt, synthetic construct
  source 1..20: mol_type = other RNA
aatcccagggccaggaaaaa

SEQ ID NO: 20381 - RNA, 20 nt, synthetic construct
  source 1..20: mol_type = other RNA
ctgcacctaatcccagggcc

SEQ ID NO: 20382 - RNA, 20 nt, synthetic construct
  source 1..20: mol_type = other RNA
cacggctgcacctaatccca

SEQ ID NO: 20383 - RNA, 20 nt, synthetic construct
  source 1..20: mol_type = other RNA
acacggctgcacctaatccc

SEQ ID NO: 20384 - RNA, 20 nt, synthetic construct
  source 1..20: mol_type = other RNA
ggtgcagccgtgttaaggag

SEQ ID NO: 20385 - RNA, 20 nt, synthetic construct
  source 1..20: mol_type = other RNA
ttaaggagaggacattcgag

SEQ ID NO: 20386 - RNA, 20 nt, synthetic construct
  source 1..20: mol_type = other RNA
taaggagaggacattcgaga

SEQ ID NO: 20387 - RNA, 20 nt, synthetic construct
  source 1..20: mol_type = other RNA
agaggacattcgagagggcg

SEQ ID NO: 20388 - RNA, 20 nt, synthetic construct
  source 1..20: mol_type = other RNA
gagggcgtggcgaagtgaag

SEQ ID NO: 20389 - RNA, 20 nt, synthetic construct
  source 1..20: mol_type = other RNA
aggaacctcacgccactgcc

SEQ ID NO: 20390 - RNA, 20 nt, synthetic construct
  source 1..20: mol_type = other RNA
cacgccactgcctggagctc

SEQ ID NO: 20391 - RNA, 20 nt, synthetic construct
  source 1..20: mol_type = other RNA
gagctccaggcagtggcgtg

SEQ ID NO: 20392 - RNA, 20 nt, synthetic construct
  source 1..20: mol_type = other RNA
gccactgcctggagctccgg

SEQ ID NO: 20393 - RNA, 20 nt, synthetic construct
  source 1..20: mol_type = other RNA
ccactgcctggagctccggt

SEQ ID NO: 20394 - RNA, 20 nt, synthetic construct
  source 1..20: mol_type = other RNA
cccaccggagctccaggcag

SEQ ID NO: 20395 - RNA, 20 nt, synthetic construct
  source 1..20: mol_type = other RNA
cctggagctccggtgggtct

SEQ ID NO: 20396 - RNA, 20 nt, synthetic construct
  source 1..20: mol_type = other RNA
agctccggtgggtctgggtc

SEQ ID NO: 20397 - RNA, 20 nt, synthetic construct
  source 1..20: mol_type = other RNA
atgaccagacccagacccac

SEQ ID NO: 20398 - RNA, 20 nt, synthetic construct
  source 1..20: mol_type = other RNA
gggtctggtcattgtctcgc

SEQ ID NO: 20399 - RNA, 20 nt, synthetic construct
  source 1..20: mol_type = other RNA
tccactctgaccactgtccc

SEQ ID NO: 20400 - RNA, 20 nt, synthetic construct
  source 1..20: mol_type = other RNA
ggacagtggtcagagtggac

SEQ ID NO: 20401 - RNA, 20 nt, synthetic construct
  source 1..20: mol_type = other RNA
gccagggacagtggtcagag

SEQ ID NO: 20402 - RNA, 20 nt, synthetic construct
  source 1..20: mol_type = other RNA
gggcagggggccagggacag

SEQ ID NO: 20403 - RNA, 20 nt, synthetic construct
  source 1..20: mol_type = other RNA
ctggacagggcagggggcca

SEQ ID NO: 20404 - RNA, 20 nt, synthetic construct
  source 1..20: mol_type = other RNA
actggacagggcagggggcc

SEQ ID NO: 20405 - RNA, 20 nt, synthetic construct
  source 1..20: mol_type = other RNA
ctgccctgtccagtccttcc

SEQ ID NO: 20406 - RNA, 20 nt, synthetic construct
  source 1..20: mol_type = other RNA
gaaggactggacagggcagg

SEQ ID NO: 20407 - RNA, 20 nt, synthetic construct
  source 1..20: mol_type = other RNA
ggaaggactggacagggcag

SEQ ID NO: 20408 - RNA, 20 nt, synthetic construct
  source 1..20: mol_type = other RNA
tggaaggactggacagggca

SEQ ID NO: 20409 - RNA, 20 nt, synthetic construct
  source 1..20: mol_type = other RNA
ctggaaggactggacagggc

SEQ ID NO: 20410 - RNA, 20 nt, synthetic construct
  source 1..20: mol_type = other RNA
ggacctggaaggactggaca

SEQ ID NO: 20411 - RNA, 20 nt, synthetic construct
  source 1..20: mol_type = other RNA
tggacctggaaggactggac

SEQ ID NO: 20412 - RNA, 20 nt, synthetic construct
  source 1..20: mol_type = other RNA
tcagatggacctggaaggac

SEQ ID NO: 20413 - RNA, 20 nt, synthetic construct
  source 1..20: mol_type = other RNA
cacactcagatggacctgga

SEQ ID NO: 20414 - RNA, 20 nt, synthetic construct
  source 1..20: mol_type = other RNA
cacacacactcagatggacc

SEQ ID NO: 20415 - RNA, 20 nt, synthetic construct
  source 1..20: mol_type = other RNA
cacacacacacacactcaga

SEQ ID NO: 20416 - RNA, 20 nt, synthetic construct
  source 1..20: mol_type = other RNA
caagtacggctgccgaacca

SEQ ID NO: 20417 - RNA, 20 nt, synthetic construct
  source 1..20: mol_type = other RNA
tcggcagccgtacttgcatt

SEQ ID NO: 20418 - RNA, 20 nt, synthetic construct
  source 1..20: mol_type = other RNA
cggcagccgtacttgcattt

SEQ ID NO: 20419 - RNA, 20 nt, synthetic construct
  source 1..20: mol_type = other RNA
acttgcatttgggcattcct

SEQ ID NO: 20420 - RNA, 20 nt, synthetic construct
  source 1..20: mol_type = other RNA
ggaatgcccaaatgcaagta

SEQ ID NO: 20421 - RNA, 20 nt, synthetic construct
  source 1..20: mol_type = other RNA
ggacacacaggagctgacct

SEQ ID NO: 20422 - RNA, 20 nt, synthetic construct
  source 1..20: mol_type = other RNA
tcagctaactgtggacacac

SEQ ID NO: 20423 - RNA, 20 nt, synthetic construct
  source 1..20: mol_type = other RNA
cttcagggttcagctaactg

SEQ ID NO: 20424 - RNA, 20 nt, synthetic construct
  source 1..20: mol_type = other RNA
gcgtcagagtgcgggcttca

SEQ ID NO: 20425 - RNA, 20 nt, synthetic construct
  source 1..20: mol_type = other RNA
agcgtcagagtgcgggcttc

SEQ ID NO: 20426 - RNA, 20 nt, synthetic construct
  source 1..20: mol_type = other RNA
gaacaggagcgtcagagtgc

SEQ ID NO: 20427 - RNA, 20 nt, synthetic construct
  source 1..20: mol_type = other RNA
agaacaggagcgtcagagtg

SEQ ID NO: 20428 - RNA, 20 nt, synthetic construct
  source 1..20: mol_type = other RNA
ctgtggagagtggagagaac

SEQ ID NO: 20429 - RNA, 20 nt, synthetic construct
  source 1..20: mol_type = other RNA
tctccacagccttagccccg

SEQ ID NO: 20430 - RNA, 20 nt, synthetic construct
  source 1..20: mol_type = other RNA
ctccacagccttagccccgt

SEQ ID NO: 20431 - RNA, 20 nt, synthetic construct
  source 1..20: mol_type = other RNA
ggcccacggggctaaggctg

SEQ ID NO: 20432 - RNA, 20 nt, synthetic construct
  source 1..20: mol_type = other RNA
ccttagccccgtgggcccca

SEQ ID NO: 20433 - RNA, 20 nt, synthetic construct
  source 1..20: mol_type = other RNA
ccgtggggcccacggggcta

SEQ ID NO: 20434 - RNA, 20 nt, synthetic construct
  source 1..20: mol_type = other RNA
cgtgggccccacggagtgag

SEQ ID NO: 20435 - RNA, 20 nt, synthetic construct
  source 1..20: mol_type = other RNA
ctcactccgtggggcccacg

SEQ ID NO: 20436 - RNA, 20 nt, synthetic construct
  source 1..20: mol_type = other RNA
gctcactccgtggggcccac

SEQ ID NO: 20437 - RNA, 20 nt, synthetic construct
  source 1..20: mol_type = other RNA
cgctcactccgtggggccca

SEQ ID NO: 20438 - RNA, 20 nt, synthetic construct
  source 1..20: mol_type = other RNA
tgcatgccgctcactccgtg

SEQ ID NO: 20439 - RNA, 20 nt, synthetic construct
  source 1..20: mol_type = other RNA
ctgcatgccgctcactccgt

SEQ ID NO: 20440 - RNA, 20 nt, synthetic construct
  source 1..20: mol_type = other RNA
gctgcatgccgctcactccg

SEQ ID NO: 20441 - RNA, 20 nt, synthetic construct
  source 1..20: mol_type = other RNA
tgagcggcatgcagcacccc

SEQ ID NO: 20442 - RNA, 20 nt, synthetic construct
  source 1..20: mol_type = other RNA
gagcggcatgcagcaccccc

SEQ ID NO: 20443 - RNA, 20 nt, synthetic construct
  source 1..20: mol_type = other RNA
cgggcctgtccagtgtcctc

SEQ ID NO: 20444 - RNA, 20 nt, synthetic construct
  source 1..20: mol_type = other RNA
aggacactggacaggcccgg

SEQ ID NO: 20445 - RNA, 20 nt, synthetic construct
  source 1..20: mol_type = other RNA
gaggacactggacaggcccg

SEQ ID NO: 20446 - RNA, 20 nt, synthetic construct
  source 1..20: mol_type = other RNA
agaggacactggacaggccc

SEQ ID NO: 20447 - RNA, 20 nt, synthetic construct
  source 1..20: mol_type = other RNA
cagaggacactggacaggcc

SEQ ID NO: 20448 - RNA, 20 nt, synthetic construct
  source 1..20: mol_type = other RNA
caggccagaggacactggac

SEQ ID NO: 20449 - RNA, 20 nt, synthetic construct
  source 1..20: mol_type = other RNA
ggcagcaggccagaggacac

SEQ ID NO: 20450 - RNA, 20 nt, synthetic construct
  source 1..20: mol_type = other RNA
ggtgcagggcagcaggccag

SEQ ID NO: 20451 - RNA, 20 nt, synthetic construct
  source 1..20: mol_type = other RNA
tgctgccctgcacccccaga

SEQ ID NO: 20452 - RNA, 20 nt, synthetic construct
  source 1..20: mol_type = other RNA
ttctgggggtgcagggcagc

SEQ ID NO: 20453 - RNA, 20 nt, synthetic construct
  source 1..20: mol_type = other RNA
cagggccttctgggggtgca

SEQ ID NO: 20454 - RNA, 20 nt, synthetic construct
  source 1..20: mol_type = other RNA
tcagggccttctgggggtgc

SEQ ID NO: 20455 - RNA, 20 nt, synthetic construct
  source 1..20: mol_type = other RNA
cccagaaggccctgacgccc

SEQ ID NO: 20456 - RNA, 20 nt, synthetic construct
  source 1..20: mol_type = other RNA
ccagaaggccctgacgccct

SEQ ID NO: 20457 - RNA, 20 nt, synthetic construct
  source 1..20: mol_type = other RNA
cagaaggccctgacgccctg

SEQ ID NO: 20458 - RNA, 20 nt, synthetic construct
  source 1..20: mol_type = other RNA
agggcgtcagggccttctgg

SEQ ID NO: 20459 - RNA, 20 nt, synthetic construct
  source 1..20: mol_type = other RNA
cagggcgtcagggccttctg

SEQ ID NO: 20460 - RNA, 20 nt, synthetic construct
  source 1..20: mol_type = other RNA
ccagggcgtcagggccttct

SEQ ID NO: 20461 - RNA, 20 nt, synthetic construct
  source 1..20: mol_type = other RNA
cccagggcgtcagggccttc

SEQ ID NO: 20462 - RNA, 20 nt, synthetic construct
  source 1..20: mol_type = other RNA
agaagtgccccagggcgtca

SEQ ID NO: 20463 - RNA, 20 nt, synthetic construct
  source 1..20: mol_type = other RNA
cagaagtgccccagggcgtc

SEQ ID NO: 20464 - RNA, 20 nt, synthetic construct
  source 1..20: mol_type = other RNA
ggggcacttctgctctgcac

SEQ ID NO: 20465 - RNA, 20 nt, synthetic construct
  source 1..20: mol_type = other RNA
tgcagagcagaagtgcccca

SEQ ID NO: 20466 - RNA, 20 nt, synthetic construct
  source 1..20: mol_type = other RNA
gtgcagagcagaagtgcccc

SEQ ID NO: 20467 - RNA, 20 nt, synthetic construct
  source 1..20: mol_type = other RNA
ctgctctgcacaggaccacg

SEQ ID NO: 20468 - RNA, 20 nt, synthetic construct
  source 1..20: mol_type = other RNA
tgctctgcacaggaccacgc

SEQ ID NO: 20469 - RNA, 20 nt, synthetic construct
  source 1..20: mol_type = other RNA
gctctgcacaggaccacgcg

SEQ ID NO: 20470 - RNA, 20 nt, synthetic construct
  source 1..20: mol_type = other RNA
ctctgcacaggaccacgcgg

SEQ ID NO: 20471 - RNA, 20 nt, synthetic construct
  source 1..20: mol_type = other RNA
gaccacgcgggggtttgcca

SEQ ID NO: 20472 - RNA, 20 nt, synthetic construct
  source 1..20: mol_type = other RNA
caccatggcaaacccccgcg

SEQ ID NO: 20473 - RNA, 20 nt, synthetic construct
  source 1..20: mol_type = other RNA
ggtttgccatggtgacataa

SEQ ID NO: 20474 - RNA, 20 nt, synthetic construct
  source 1..20: mol_type = other RNA
gtttgccatggtgacataaa

SEQ ID NO: 20475 - RNA, 20 nt, synthetic construct
  source 1..20: mol_type = other RNA
tttgccatggtgacataaag

SEQ ID NO: 20476 - RNA, 20 nt, synthetic construct
  source 1..20: mol_type = other RNA
catggtgacataaaggggcg

SEQ ID NO: 20477 - RNA, 20 nt, synthetic construct
  source 1..20: mol_type = other RNA
ggtgacataaaggggcgcgg

SEQ ID NO: 20478 - RNA, 20 nt, synthetic construct
  source 1..20: mol_type = other RNA
cgcgcccctttatgtcacca

SEQ ID NO: 20479 - RNA, 20 nt, synthetic construct
  source 1..20: mol_type = other RNA
acataaaggggcgcggagga

SEQ ID NO: 20480 - RNA, 20 nt, synthetic construct
  source 1..20: mol_type = other RNA
aaaggggcgcggaggaagga

SEQ ID NO: 20481 - RNA, 20 nt, synthetic construct
  source 1..20: mol_type = other RNA
gaaggagcgtgaccagcctg

SEQ ID NO: 20482 - RNA, 20 nt, synthetic construct
  source 1..20: mol_type = other RNA
cagcctgtggactgcgcccc

SEQ ID NO: 20483 - RNA, 20 nt, synthetic construct
  source 1..20: mol_type = other RNA
caggggcgcagtccacaggc

SEQ ID NO: 20484 - RNA, 20 nt, synthetic construct
  source 1..20: mol_type = other RNA
tgtggactgcgcccctggct

SEQ ID NO: 20485 - RNA, 20 nt, synthetic construct
  source 1..20: mol_type = other RNA
cagccaggggcgcagtccac

SEQ ID NO: 20486 - RNA, 20 nt, synthetic construct
  source 1..20: mol_type = other RNA
tgcgcccctggctgggagga

SEQ ID NO: 20487 - RNA, 20 nt, synthetic construct
  source 1..20: mol_type = other RNA
ccctggctgggaggaaggac

SEQ ID NO: 20488 - RNA, 20 nt, synthetic construct
  source 1..20: mol_type = other RNA
cctggctgggaggaaggact

SEQ ID NO: 20489 - RNA, 20 nt, synthetic construct
  source 1..20: mol_type = other RNA
ctggctgggaggaaggactg

SEQ ID NO: 20490 - RNA, 20 nt, synthetic construct
  source 1..20: mol_type = other RNA
tggctgggaggaaggactgg

SEQ ID NO: 20491 - RNA, 20 nt, synthetic construct
  source 1..20: mol_type = other RNA
cagtccttcctcccagccag

SEQ ID NO: 20492 - RNA, 20 nt, synthetic construct
  source 1..20: mol_type = other RNA
ccagtccttcctcccagcca

SEQ ID NO: 20493 - RNA, 20 nt, synthetic construct
  source 1..20: mol_type = other RNA
cccagtccttcctcccagcc

SEQ ID NO: 20494 - RNA, 20 nt, synthetic construct
  source 1..20: mol_type = other RNA
gcactgggagtggaggatct

SEQ ID NO: 20495 - RNA, 20 nt, synthetic construct
  source 1..20: mol_type = other RNA
ggcactgggagtggaggatc

SEQ ID NO: 20496 - RNA, 20 nt, synthetic construct
  source 1..20: mol_type = other RNA
tccactcccagtgccccaca

SEQ ID NO: 20497 - RNA, 20 nt, synthetic construct
  source 1..20: mol_type = other RNA
ccactcccagtgccccacaa

SEQ ID NO: 20498 - RNA, 20 nt, synthetic construct
  source 1..20: mol_type = other RNA
ttgtggggcactgggagtgg

SEQ ID NO: 20499 - RNA, 20 nt, synthetic construct
  source 1..20: mol_type = other RNA
cccttgtggggcactgggag

SEQ ID NO: 20500 - RNA, 20 nt, synthetic construct
  source 1..20: mol_type = other RNA
cgacgcccttgtggggcact

SEQ ID NO: 20501 - RNA, 20 nt, synthetic construct
  source 1..20: mol_type = other RNA
gcgacgcccttgtggggcac

SEQ ID NO: 20502 - RNA, 20 nt, synthetic construct
  source 1..20: mol_type = other RNA
taggaagcgacgcccttgtg

SEQ ID NO: 20503 - RNA, 20 nt, synthetic construct
  source 1..20: mol_type = other RNA
ttaggaagcgacgcccttgt

SEQ ID NO: 20504 - RNA, 20 nt, synthetic construct
  source 1..20: mol_type = other RNA
cttaggaagcgacgcccttg

SEQ ID NO: 20505 - RNA, 20 nt, synthetic construct
  source 1..20: mol_type = other RNA
ctaagtctctgtgaatttgt

SEQ ID NO: 20506 - RNA, 20 nt, synthetic construct
  source 1..20: mol_type = other RNA
caacaaattcacagagactt

SEQ ID NO: 20507 - RNA, 20 nt, synthetic construct
  source 1..20: mol_type = other RNA
tctgtgaatttgttggtcag

SEQ ID NO: 20508 - RNA, 20 nt, synthetic construct
  source 1..20: mol_type = other RNA
ttctcgtgtctcctcctgtg

SEQ ID NO: 20509 - RNA, 20 nt, synthetic construct
  source 1..20: mol_type = other RNA
tctcgtgtctcctcctgtgt

SEQ ID NO: 20510 - RNA, 20 nt, synthetic construct
  source 1..20: mol_type = other RNA
ctcgtgtctcctcctgtgtg

SEQ ID NO: 20511 - RNA, 20 nt, synthetic construct
  source 1..20: mol_type = other RNA
tctcctcctgtgtggggcct

SEQ ID NO: 20512 - RNA, 20 nt, synthetic construct
  source 1..20: mol_type = other RNA
ctcctcctgtgtggggcctt

SEQ ID NO: 20513 - RNA, 20 nt, synthetic construct
  source 1..20: mol_type = other RNA
tcctcctgtgtggggccttg

SEQ ID NO: 20514 - RNA, 20 nt, synthetic construct
  source 1..20: mol_type = other RNA
accccaaggccccacacagg

SEQ ID NO: 20515 - RNA, 20 nt, synthetic construct
  source 1..20: mol_type = other RNA
tgtggggccttggggtagcc

SEQ ID NO: 20516 - RNA, 20 nt, synthetic construct
  source 1..20: mol_type = other RNA
gtggggccttggggtagcca

SEQ ID NO: 20517 - RNA, 20 nt, synthetic construct
  source 1..20: mol_type = other RNA
ggccttggggtagccagggc

SEQ ID NO: 20518 - RNA, 20 nt, synthetic construct
  source 1..20: mol_type = other RNA
ttggggtagccagggcaggc

SEQ ID NO: 20519 - RNA, 20 nt, synthetic construct
  source 1..20: mol_type = other RNA
tggggtagccagggcaggcc

SEQ ID NO: 20520 - RNA, 20 nt, synthetic construct
  source 1..20: mol_type = other RNA
ggcctgccctggctacccca

SEQ ID NO: 20521 - RNA, 20 nt, synthetic construct
  source 1..20: mol_type = other RNA
gccagggcaggccgggcctc

SEQ ID NO: 20522 - RNA, 20 nt, synthetic construct
  source 1..20: mol_type = other RNA
agggcaggccgggcctccgg

SEQ ID NO: 20523 - RNA, 20 nt, synthetic construct
  source 1..20: mol_type = other RNA
accggaggcccggcctgccc

SEQ ID NO: 20524 - RNA, 20 nt, synthetic construct
  source 1..20: mol_type = other RNA
ggccgggcctccggtggcca

SEQ ID NO: 20525 - RNA, 20 nt, synthetic construct
  source 1..20: mol_type = other RNA
gcctccggtggccaaggtct

SEQ ID NO: 20526 - RNA, 20 nt, synthetic construct
  source 1..20: mol_type = other RNA
gaccttggccaccggaggcc

SEQ ID NO: 20527 - RNA, 20 nt, synthetic construct
  source 1..20: mol_type = other RNA
tccggtggccaaggtctcgg

SEQ ID NO: 20528 - RNA, 20 nt, synthetic construct
  source 1..20: mol_type = other RNA
tccgagaccttggccaccgg

SEQ ID NO: 20529 - RNA, 20 nt, synthetic construct
  source 1..20: mol_type = other RNA
tggccaaggtctcggaggcc

SEQ ID NO: 20530 - RNA, 20 nt, synthetic construct
  source 1..20: mol_type = other RNA
gcctccgagaccttggccac

SEQ ID NO: 20531 - RNA, 20 nt, synthetic construct
  source 1..20: mol_type = other RNA
catcctggcctccgagacct

SEQ ID NO: 20532 - RNA, 20 nt, synthetic construct
  source 1..20: mol_type = other RNA
ggaggccaggatgcctgccc

SEQ ID NO: 20533 - RNA, 20 nt, synthetic construct
  source 1..20: mol_type = other RNA
gcatgccagggcaggcatcc

SEQ ID NO: 20534 - RNA, 20 nt, synthetic construct
  source 1..20: mol_type = other RNA
tgcctgccctggcatgcctc

SEQ ID NO: 20535 - RNA, 20 nt, synthetic construct
  source 1..20: mol_type = other RNA
ctgccctggcatgcctccgg

SEQ ID NO: 20536 - RNA, 20 nt, synthetic construct
  source 1..20: mol_type = other RNA
ctccggaggcatgccagggc

SEQ ID NO: 20537 - RNA, 20 nt, synthetic construct
  source 1..20: mol_type = other RNA
cagcctccggaggcatgcca

SEQ ID NO: 20538 - RNA, 20 nt, synthetic construct
  source 1..20: mol_type = other RNA
catgcctccggaggctgtgt

SEQ ID NO: 20539 - RNA, 20 nt, synthetic construct
  source 1..20: mol_type = other RNA
cgtgccgacacagcctccgg

SEQ ID NO: 20540 - RNA, 20 nt, synthetic construct
  source 1..20: mol_type = other RNA
acacgtgccgacacagcctc

SEQ ID NO: 20541 - RNA, 20 nt, synthetic construct
  source 1..20: mol_type = other RNA
gtgtcggcacgtgtccccgc

SEQ ID NO: 20542 - RNA, 20 nt, synthetic construct
  source 1..20: mol_type = other RNA
caggaaaaggacagcctgcg

SEQ ID NO: 20543 - RNA, 20 nt, synthetic construct
  source 1..20: mol_type = other RNA
gcaggaaaaggacagcctgc

SEQ ID NO: 20544 - RNA, 20 nt, synthetic construct
  source 1..20: mol_type = other RNA
agcaggaaaaggacagcctg

SEQ ID NO: 20545 - RNA, 20 nt, synthetic construct
  source 1..20: mol_type = other RNA
agaagatgaacagcaggaaa

SEQ ID NO: 20546 - RNA, 20 nt, synthetic construct
  source 1..20: mol_type = other RNA
acaggcagaagatgaacagc

SEQ ID NO: 20547 - RNA, 20 nt, synthetic construct
  source 1..20: mol_type = other RNA
cctgttcagcgttttcatct

SEQ ID NO: 20548 - RNA, 20 nt, synthetic construct
  source 1..20: mol_type = other RNA
ccgagatgaaaacgctgaac

SEQ ID NO: 20549 - RNA, 20 nt, synthetic construct
  source 1..20: mol_type = other RNA
atctcggcctactacctata

SEQ ID NO: 20550 - RNA, 20 nt, synthetic construct
  source 1..20: mol_type = other RNA
cggcctactacctatatggc

SEQ ID NO: 20551 - RNA, 20 nt, synthetic construct
  source 1..20: mol_type = other RNA
cttccagccatataggtagt

SEQ ID NO: 20552 - RNA, 20 nt, synthetic construct
  source 1..20: mol_type = other RNA
atatggctggaagcgaggcc

SEQ ID NO: 20553 - RNA, 20 nt, synthetic construct
  source 1..20: mol_type = other RNA
ggcctcgcttccagccatat

SEQ ID NO: 20554 - RNA, 20 nt, synthetic construct
  source 1..20: mol_type = other RNA
gaagcgaggcctggagccct

SEQ ID NO: 20555 - RNA, 20 nt, synthetic construct
  source 1..20: mol_type = other RNA
gcgaggcctggagccctcgg

SEQ ID NO: 20556 - RNA, 20 nt, synthetic construct
  source 1..20: mol_type = other RNA
gggcatccgccgagggctcc

SEQ ID NO: 20557 - RNA, 20 nt, synthetic construct
  source 1..20: mol_type = other RNA
ggctcgggggcatccgccga

SEQ ID NO: 20558 - RNA, 20 nt, synthetic construct
  source 1..20: mol_type = other RNA
aggctcgggggcatccgccg

SEQ ID NO: 20559 - RNA, 20 nt, synthetic construct
  source 1..20: mol_type = other RNA
gatgcccccgagcctgactg

SEQ ID NO: 20560 - RNA, 20 nt, synthetic construct
  source 1..20: mol_type = other RNA
atgcccccgagcctgactgc

SEQ ID NO: 20561 - RNA, 20 nt, synthetic construct
  source 1..20: mol_type = other RNA
tgcccccgagcctgactgcg

SEQ ID NO: 20562 - RNA, 20 nt, synthetic construct
  source 1..20: mol_type = other RNA
gtccccgcagtcaggctcgg

SEQ ID NO: 20563 - RNA, 20 nt, synthetic construct
  source 1..20: mol_type = other RNA
ggtccccgcagtcaggctcg

SEQ ID NO: 20564 - RNA, 20 nt, synthetic construct
  source 1..20: mol_type = other RNA
gggtccccgcagtcaggctc

SEQ ID NO: 20565 - RNA, 20 nt, synthetic construct
  source 1..20: mol_type = other RNA
cgggtccccgcagtcaggct

SEQ ID NO: 20566 - RNA, 20 nt, synthetic construct
  source 1..20: mol_type = other RNA
ggcggcgggtccccgcagtc

SEQ ID NO: 20567 - RNA, 20 nt, synthetic construct
  source 1..20: mol_type = other RNA
gactgggggccacaggcggc

SEQ ID NO: 20568 - RNA, 20 nt, synthetic construct
  source 1..20: mol_type = other RNA
cgactgggggccacaggcgg

SEQ ID NO: 20569 - RNA, 20 nt, synthetic construct
  source 1..20: mol_type = other RNA
aggcgactgggggccacagg

SEQ ID NO: 20570 - RNA, 20 nt, synthetic construct
  source 1..20: mol_type = other RNA
agcaggcgactgggggccac

SEQ ID NO: 20571 - RNA, 20 nt, synthetic construct
  source 1..20: mol_type = other RNA
gagtggcagcaggcgactgg

SEQ ID NO: 20572 - RNA, 20 nt, synthetic construct
  source 1..20: mol_type = other RNA
tgagtggcagcaggcgactg

SEQ ID NO: 20573 - RNA, 20 nt, synthetic construct
  source 1..20: mol_type = other RNA
ttgagtggcagcaggcgact

SEQ ID NO: 20574 - RNA, 20 nt, synthetic construct
  source 1..20: mol_type = other RNA
cttgagtggcagcaggcgac

SEQ ID NO: 20575 - RNA, 20 nt, synthetic construct
  source 1..20: mol_type = other RNA
gctgccactcaagcctgtgc

SEQ ID NO: 20576 - RNA, 20 nt, synthetic construct
  source 1..20: mol_type = other RNA
gcacaggcttgagtggcagc

SEQ ID NO: 20577 - RNA, 20 nt, synthetic construct
  source 1..20: mol_type = other RNA
gctgcctgcacaggcttgag

SEQ ID NO: 20578 - RNA, 20 nt, synthetic construct
  source 1..20: mol_type = other RNA
gaaggggtggctgcctgcac

SEQ ID NO: 20579 - RNA, 20 nt, synthetic construct
  source 1..20: mol_type = other RNA
cccttcccgcacagacccgt

SEQ ID NO: 20580 - RNA, 20 nt, synthetic construct
  source 1..20: mol_type = other RNA
cgggtctgtgcgggaagggg

SEQ ID NO: 20581 - RNA, 20 nt, synthetic construct
  source 1..20: mol_type = other RNA
caacgggtctgtgcgggaag

SEQ ID NO: 20582 - RNA, 20 nt, synthetic construct
  source 1..20: mol_type = other RNA
ccaacgggtctgtgcgggaa

SEQ ID NO: 20583 - RNA, 20 nt, synthetic construct
  source 1..20: mol_type = other RNA
accaacgggtctgtgcggga

SEQ ID NO: 20584 - RNA, 20 nt, synthetic construct
  source 1..20: mol_type = other RNA
cagcaccaacgggtctgtgc

SEQ ID NO: 20585 - RNA, 20 nt, synthetic construct
  source 1..20: mol_type = other RNA
ccagcaccaacgggtctgtg

SEQ ID NO: 20586 - RNA, 20 nt, synthetic construct
  source 1..20: mol_type = other RNA
cccgttggtgctggtctttg

SEQ ID NO: 20587 - RNA, 20 nt, synthetic construct
  source 1..20: mol_type = other RNA
ccacaaagaccagcaccaac

SEQ ID NO: 20588 - RNA, 20 nt, synthetic construct
  source 1..20: mol_type = other RNA
tccacaaagaccagcaccaa

SEQ ID NO: 20589 - RNA, 20 nt, synthetic construct
  source 1..20: mol_type = other RNA
ggagagcctctactcgcaac

SEQ ID NO: 20590 - RNA, 20 nt, synthetic construct
  source 1..20: mol_type = other RNA
gagagcctctactcgcaact

SEQ ID NO: 20591 - RNA, 20 nt, synthetic construct
  source 1..20: mol_type = other RNA
cctctactcgcaactgggcc

SEQ ID NO: 20592 - RNA, 20 nt, synthetic construct
  source 1..20: mol_type = other RNA
ctactcgcaactgggccagg

SEQ ID NO: 20593 - RNA, 20 nt, synthetic construct
  source 1..20: mol_type = other RNA
cctggcccagttgcgagtag

SEQ ID NO: 20594 - RNA, 20 nt, synthetic construct
  source 1..20: mol_type = other RNA
ctcgcaactgggccaggagg

SEQ ID NO: 20595 - RNA, 20 nt, synthetic construct
  source 1..20: mol_type = other RNA
gcaactgggccaggaggtgg

SEQ ID NO: 20596 - RNA, 20 nt, synthetic construct
  source 1..20: mol_type = other RNA
ccaggaggtggtggccatcc

SEQ ID NO: 20597 - RNA, 20 nt, synthetic construct
  source 1..20: mol_type = other RNA
ccaggatggccaccacctcc

SEQ ID NO: 20598 - RNA, 20 nt, synthetic construct
  source 1..20: mol_type = other RNA
gaagcggctggactccagga

SEQ ID NO: 20599 - RNA, 20 nt, synthetic construct
  source 1..20: mol_type = other RNA
atttgaagcggctggactcc

SEQ ID NO: 20600 - RNA, 20 nt, synthetic construct
  source 1..20: mol_type = other RNA
tgtgcggtatttgaagcggc

SEQ ID NO: 20601 - RNA, 20 nt, synthetic construct
  source 1..20: mol_type = other RNA
tctctgtgcggtatttgaag

SEQ ID NO: 20602 - RNA, 20 nt, synthetic construct
  source 1..20: mol_type = other RNA
ataccgcacagagattgcgc

SEQ ID NO: 20603 - RNA, 20 nt, synthetic construct
  source 1..20: mol_type = other RNA
taccgcacagagattgcgcc

SEQ ID NO: 20604 - RNA, 20 nt, synthetic construct
  source 1..20: mol_type = other RNA
cacagagattgcgccgggca

SEQ ID NO: 20605 - RNA, 20 nt, synthetic construct
  source 1..20: mol_type = other RNA
acagagattgcgccgggcaa

SEQ ID NO: 20606 - RNA, 20 nt, synthetic construct
  source 1..20: mol_type = other RNA
tgcccggcgcaatctctgtg

SEQ ID NO: 20607 - RNA, 20 nt, synthetic construct
  source 1..20: mol_type = other RNA
gtgggcatgtcacccttgcc

SEQ ID NO: 20608 - RNA, 20 nt, synthetic construct
  source 1..20: mol_type = other RNA
catgcccacgctcactgaca

SEQ ID NO: 20609 - RNA, 20 nt, synthetic construct
  source 1..20: mol_type = other RNA
atgcccacgctcactgacaa

SEQ ID NO: 20610 - RNA, 20 nt, synthetic construct
  source 1..20: mol_type = other RNA
acgctcactgacaagggccg

SEQ ID NO: 20611 - RNA, 20 nt, synthetic construct
  source 1..20: mol_type = other RNA
cggcccttgtcagtgagcgt

SEQ ID NO: 20612 - RNA, 20 nt, synthetic construct
  source 1..20: mol_type = other RNA
acggcccttgtcagtgagcg

SEQ ID NO: 20613 - RNA, 20 nt, synthetic construct
  source 1..20: mol_type = other RNA
tgatgagggcgaagcggcca

SEQ ID NO: 20614 - RNA, 20 nt, synthetic construct
  source 1..20: mol_type = other RNA
catagatgatgagggcgaag

SEQ ID NO: 20615 - RNA, 20 nt, synthetic construct
  source 1..20: mol_type = other RNA
gatgttctcatagatgatga

SEQ ID NO: 20616 - RNA, 20 nt, synthetic construct
  source 1..20: mol_type = other RNA
ggatgttctcatagatgatg

SEQ ID NO: 20617 - RNA, 20 nt, synthetic construct
  source 1..20: mol_type = other RNA
catcctcaagtatgtcaacc

SEQ ID NO: 20618 - RNA, 20 nt, synthetic construct
  source 1..20: mol_type = other RNA
agtatgtcaacctggacgcc

SEQ ID NO: 20619 - RNA, 20 nt, synthetic construct
  source 1..20: mol_type = other RNA
tcaacctggacgcctggaac

SEQ ID NO: 20620 - RNA, 20 nt, synthetic construct
  source 1..20: mol_type = other RNA
caacctggacgcctggaacc

SEQ ID NO: 20621 - RNA, 20 nt, synthetic construct
  source 1..20: mol_type = other RNA
gctcccggttccaggcgtcc

SEQ ID NO: 20622 - RNA, 20 nt, synthetic construct
  source 1..20: mol_type = other RNA
cgcctggaaccgggagctgc

SEQ ID NO: 20623 - RNA, 20 nt, synthetic construct
  source 1..20: mol_type = other RNA
gtccagcagctcccggttcc

SEQ ID NO: 20624 - RNA, 20 nt, synthetic construct
  source 1..20: mol_type = other RNA
agtacttgtccagcagctcc

SEQ ID NO: 20625 - RNA, 20 nt, synthetic construct
  source 1..20: mol_type = other RNA
gctgctggacaagtactgtg

SEQ ID NO: 20626 - RNA, 20 nt, synthetic construct
  source 1..20: mol_type = other RNA
gacaagtactgtgtggccta

SEQ ID NO: 20627 - RNA, 20 nt, synthetic construct
  source 1..20: mol_type = other RNA
gtactgtgtggcctacggcg

SEQ ID NO: 20628 - RNA, 20 nt, synthetic construct
  source 1..20: mol_type = other RNA
tactgtgtggcctacggcgt

SEQ ID NO: 20629 - RNA, 20 nt, synthetic construct
  source 1..20: mol_type = other RNA
gcctacggcgtgggcatcat

SEQ ID NO: 20630 - RNA, 20 nt, synthetic construct
  source 1..20: mol_type = other RNA
gccaatgatgcccacgccgt

SEQ ID NO: 20631 - RNA, 20 nt, synthetic construct
  source 1..20: mol_type = other RNA
gggcatcattggcttcttca

SEQ ID NO: 20632 - RNA, 20 nt, synthetic construct
  source 1..20: mol_type = other RNA
cttcaaggtacacaagaagc

SEQ ID NO: 20633 - RNA, 20 nt, synthetic construct
  source 1..20: mol_type = other RNA
ttcaaggtacacaagaagca

SEQ ID NO: 20634 - RNA, 20 nt, synthetic construct
  source 1..20: mol_type = other RNA
agggggctctgaactgctcg

SEQ ID NO: 20635 - RNA, 20 nt, synthetic construct
  source 1..20: mol_type = other RNA
gagggggctctgaactgctc

SEQ ID NO: 20636 - RNA, 20 nt, synthetic construct
  source 1..20: mol_type = other RNA
agagggggctctgaactgct

SEQ ID NO: 20637 - RNA, 20 nt, synthetic construct
  source 1..20: mol_type = other RNA
caggcactgagctgcagagg

SEQ ID NO: 20638 - RNA, 20 nt, synthetic construct
  source 1..20: mol_type = other RNA
tcaggcactgagctgcagag

SEQ ID NO: 20639 - RNA, 20 nt, synthetic construct
  source 1..20: mol_type = other RNA
ttcaggcactgagctgcaga

SEQ ID NO: 20640 - RNA, 20 nt, synthetic construct
  source 1..20: mol_type = other RNA
attcaggcactgagctgcag

SEQ ID NO: 20641 - RNA, 20 nt, synthetic construct
  source 1..20: mol_type = other RNA
tgaattctcatttgtgaaat

SEQ ID NO: 20642 - RNA, 20 nt, synthetic construct
  source 1..20: mol_type = other RNA
tatttcacaaatgagaattc

SEQ ID NO: 20643 - RNA, 20 nt, synthetic construct
  source 1..20: mol_type = other RNA
catttgtgaaataggtgtaa

SEQ ID NO: 20644 - RNA, 20 nt, synthetic construct
  source 1..20: mol_type = other RNA
taatggtagcacccgcctcc

SEQ ID NO: 20645 - RNA, 20 nt, synthetic construct
  source 1..20: mol_type = other RNA
aatggtagcacccgcctcct

SEQ ID NO: 20646 - RNA, 20 nt, synthetic construct
  source 1..20: mol_type = other RNA
atggtagcacccgcctcctg

SEQ ID NO: 20647 - RNA, 20 nt, synthetic construct
  source 1..20: mol_type = other RNA
cacccgcctcctggggttgt

SEQ ID NO: 20648 - RNA, 20 nt, synthetic construct
  source 1..20: mol_type = other RNA
acccgcctcctggggttgtt

SEQ ID NO: 20649 - RNA, 20 nt, synthetic construct
  source 1..20: mol_type = other RNA
cgcctcctggggttgttggg

SEQ ID NO: 20650 - RNA, 20 nt, synthetic construct
  source 1..20: mol_type = other RNA
gcctcctggggttgttggga

SEQ ID NO: 20651 - RNA, 20 nt, synthetic construct
  source 1..20: mol_type = other RNA
tcccaacaaccccaggaggc

SEQ ID NO: 20652 - RNA, 20 nt, synthetic construct
  source 1..20: mol_type = other RNA
ctcccaacaaccccaggagg

SEQ ID NO: 20653 - RNA, 20 nt, synthetic construct
  source 1..20: mol_type = other RNA
accctcccaacaaccccagg

SEQ ID NO: 20654 - RNA, 20 nt, synthetic construct
  source 1..20: mol_type = other RNA
ttaaccctcccaacaacccc

SEQ ID NO: 20655 - RNA, 20 nt, synthetic construct
  source 1..20: mol_type = other RNA
tattcaccaacattcatgga

SEQ ID NO: 20656 - RNA, 20 nt, synthetic construct
  source 1..20: mol_type = other RNA
atattcaccaacattcatgg

SEQ ID NO: 20657 - RNA, 20 nt, synthetic construct
  source 1..20: mol_type = other RNA
tcaatattcaccaacattca

SEQ ID NO: 20658 - RNA, 20 nt, synthetic construct
  source 1..20: mol_type = other RNA
gaatattgataccactgtta

SEQ ID NO: 20659 - RNA, 20 nt, synthetic construct
  source 1..20: mol_type = other RNA
tcacatgtggaccataacag

SEQ ID NO: 20660 - RNA, 20 nt, synthetic construct
  source 1..20: mol_type = other RNA
atgtgagagactgtgtcctt

SEQ ID NO: 20661 - RNA, 20 nt, synthetic construct
  source 1..20: mol_type = other RNA
tgtgagagactgtgtccttt

SEQ ID NO: 20662 - RNA, 20 nt, synthetic construct
  source 1..20: mol_type = other RNA
gtgagagactgtgtcctttg

SEQ ID NO: 20663 - RNA, 20 nt, synthetic construct
  source 1..20: mol_type = other RNA
gactgtgtcctttggggttc

SEQ ID NO: 20664 - RNA, 20 nt, synthetic construct
  source 1..20: mol_type = other RNA
tgtcacatccagaaccccaa

SEQ ID NO: 20665 - RNA, 20 nt, synthetic construct
  source 1..20: mol_type = other RNA
tcctgccctccattgactgc

SEQ ID NO: 20666 - RNA, 20 nt, synthetic construct
  source 1..20: mol_type = other RNA
cagtcaatggagggcaggaa

SEQ ID NO: 20667 - RNA, 20 nt, synthetic construct
  source 1..20: mol_type = other RNA
gcagtcaatggagggcagga

SEQ ID NO: 20668 - RNA, 20 nt, synthetic construct
  source 1..20: mol_type = other RNA
gcctgcagtcaatggagggc

SEQ ID NO: 20669 - RNA, 20 nt, synthetic construct
  source 1..20: mol_type = other RNA
attggcctgcagtcaatgga

SEQ ID NO: 20670 - RNA, 20 nt, synthetic construct
  source 1..20: mol_type = other RNA
cattggcctgcagtcaatgg

SEQ ID NO: 20671 - RNA, 20 nt, synthetic construct
  source 1..20: mol_type = other RNA
tctcattggcctgcagtcaa

SEQ ID NO: 20672 - RNA, 20 nt, synthetic construct
  source 1..20: mol_type = other RNA
actcagcaggctgttctcat

SEQ ID NO: 20673 - RNA, 20 nt, synthetic construct
  source 1..20: mol_type = other RNA
cctgctgagtgcgcagctca

SEQ ID NO: 20674 - RNA, 20 nt, synthetic construct
  source 1..20: mol_type = other RNA
ctgctgagtgcgcagctcaa

SEQ ID NO: 20675 - RNA, 20 nt, synthetic construct
  source 1..20: mol_type = other RNA
ccttgagctgcgcactcagc

SEQ ID NO: 20676 - RNA, 20 nt, synthetic construct
  source 1..20: mol_type = other RNA
cctgttcctgcactcaaacc

SEQ ID NO: 20677 - RNA, 20 nt, synthetic construct
  source 1..20: mol_type = other RNA
ctgttcctgcactcaaacct

SEQ ID NO: 20678 - RNA, 20 nt, synthetic construct
  source 1..20: mol_type = other RNA
ggtttgagtgcaggaacagg

SEQ ID NO: 20679 - RNA, 20 nt, synthetic construct
  source 1..20: mol_type = other RNA
aggtttgagtgcaggaacag

SEQ ID NO: 20680 - RNA, 20 nt, synthetic construct
  source 1..20: mol_type = other RNA
caggtttgagtgcaggaaca

SEQ ID NO: 20681 - RNA, 20 nt, synthetic construct
  source 1..20: mol_type = other RNA
ccaggtttgagtgcaggaac

SEQ ID NO: 20682 - RNA, 20 nt, synthetic construct
  source 1..20: mol_type = other RNA
gcactcaaacctgggcctga

SEQ ID NO: 20683 - RNA, 20 nt, synthetic construct
  source 1..20: mol_type = other RNA
tcaggcccaggtttgagtgc

SEQ ID NO: 20684 - RNA, 20 nt, synthetic construct
  source 1..20: mol_type = other RNA
tgctgcagtccttcaggccc

SEQ ID NO: 20685 - RNA, 20 nt, synthetic construct
  source 1..20: mol_type = other RNA
ggttgatgctgcagtccttc

SEQ ID NO: 20686 - RNA, 20 nt, synthetic construct
  source 1..20: mol_type = other RNA
cgtagagcagcggggacttg

SEQ ID NO: 20687 - RNA, 20 nt, synthetic construct
  source 1..20: mol_type = other RNA
acgtagagcagcggggactt

SEQ ID NO: 20688 - RNA, 20 nt, synthetic construct
  source 1..20: mol_type = other RNA
cacgtagagcagcggggact

SEQ ID NO: 20689 - RNA, 20 nt, synthetic construct
  source 1..20: mol_type = other RNA
tcgcgtcacgtagagcagcg

SEQ ID NO: 20690 - RNA, 20 nt, synthetic construct
  source 1..20: mol_type = other RNA
gtcgcgtcacgtagagcagc

SEQ ID NO: 20691 - RNA, 20 nt, synthetic construct
  source 1..20: mol_type = other RNA
ggtcgcgtcacgtagagcag

SEQ ID NO: 20692 - RNA, 20 nt, synthetic construct
  source 1..20: mol_type = other RNA
ctacgtgacgcgacctagcg

SEQ ID NO: 20693 - RNA, 20 nt, synthetic construct
  source 1..20: mol_type = other RNA
cgtgacgcgacctagcgagg

SEQ ID NO: 20694 - RNA, 20 nt, synthetic construct
  source 1..20: mol_type = other RNA
cgacctagcgaggtggagaa

SEQ ID NO: 20695 - RNA, 20 nt, synthetic construct
  source 1..20: mol_type = other RNA
acacctttctccacctcgct

SEQ ID NO: 20696 - RNA, 20 nt, synthetic construct
  source 1..20: mol_type = other RNA
gtggagaaaggtgtgctccc

SEQ ID NO: 20697 - RNA, 20 nt, synthetic construct
  source 1..20: mol_type = other RNA
gaaaggtgtgctccccggcg

SEQ ID NO: 20698 - RNA, 20 nt, synthetic construct
  source 1..20: mol_type = other RNA
gtgtgctccccggcgaggac

SEQ ID NO: 20699 - RNA, 20 nt, synthetic construct
  source 1..20: mol_type = other RNA
gctccccggcgaggactgga

SEQ ID NO: 20700 - RNA, 20 nt, synthetic construct
  source 1..20: mol_type = other RNA
aaaccgtccagtcctcgccg

SEQ ID NO: 20701 - RNA, 20 nt, synthetic construct
  source 1..20: mol_type = other RNA
aaaaccgtccagtcctcgcc

SEQ ID NO: 20702 - RNA, 20 nt, synthetic construct
  source 1..20: mol_type = other RNA
gaaaaccgtccagtcctcgc

SEQ ID NO: 20703 - RNA, 20 nt, synthetic construct
  source 1..20: mol_type = other RNA
cataggtggagtgatttgac

SEQ ID NO: 20704 - RNA, 20 nt, synthetic construct
  source 1..20: mol_type = other RNA
cacctatgagccagtgctgc

SEQ ID NO: 20705 - RNA, 20 nt, synthetic construct
  source 1..20: mol_type = other RNA
cagcagcactggctcatagg

SEQ ID NO: 20706 - RNA, 20 nt, synthetic construct
  source 1..20: mol_type = other RNA
ggccagcagcactggctcat

SEQ ID NO: 20707 - RNA, 20 nt, synthetic construct
  source 1..20: mol_type = other RNA
cgcgtcttggccagcagcac

SEQ ID NO: 20708 - RNA, 20 nt, synthetic construct
  source 1..20: mol_type = other RNA
ggactcagacgagcgcgtct

SEQ ID NO: 20709 - RNA, 20 nt, synthetic construct
  source 1..20: mol_type = other RNA
gtctgagtccatcccacacc

SEQ ID NO: 20710 - RNA, 20 nt, synthetic construct
  source 1..20: mol_type = other RNA
tctgagtccatcccacacct

SEQ ID NO: 20711 - RNA, 20 nt, synthetic construct
  source 1..20: mol_type = other RNA
gtctgcgcccaggtgtggga

SEQ ID NO: 20712 - RNA, 20 nt, synthetic construct
  source 1..20: mol_type = other RNA
cggcgtctgcgcccaggtgt

SEQ ID NO: 20713 - RNA, 20 nt, synthetic construct
  source 1..20: mol_type = other RNA
ccggcgtctgcgcccaggtg

SEQ ID NO: 20714 - RNA, 20 nt, synthetic construct
  source 1..20: mol_type = other RNA
gcaggccggcgtctgcgccc

SEQ ID NO: 20715 - RNA, 20 nt, synthetic construct
  source 1..20: mol_type = other RNA
gtgcagtgcagcatgcaggc

SEQ ID NO: 20716 - RNA, 20 nt, synthetic construct
  source 1..20: mol_type = other RNA
tggcgtgcagtgcagcatgc

SEQ ID NO: 20717 - RNA, 20 nt, synthetic construct
  source 1..20: mol_type = other RNA
tgctgcactgcacgccactg

SEQ ID NO: 20718 - RNA, 20 nt, synthetic construct
  source 1..20: mol_type = other RNA
actgcacgccactgtggtcc

SEQ ID NO: 20719 - RNA, 20 nt, synthetic construct
  source 1..20: mol_type = other RNA
cgccactgtggtccaggacc

SEQ ID NO: 20720 - RNA, 20 nt, synthetic construct
  source 1..20: mol_type = other RNA
gccactgtggtccaggacct

SEQ ID NO: 20721 - RNA, 20 nt, synthetic construct
  source 1..20: mol_type = other RNA
gcccaggtcctggaccacag

SEQ ID NO: 20722 - RNA, 20 nt, synthetic construct
  source 1..20: mol_type = other RNA
caggacctgggcctgcacga

SEQ ID NO: 20723 - RNA, 20 nt, synthetic construct
  source 1..20: mol_type = other RNA
cgtcgtgcaggcccaggtcc

SEQ ID NO: 20724 - RNA, 20 nt, synthetic construct
  source 1..20: mol_type = other RNA
ggatgccgtcgtgcaggccc

SEQ ID NO: 20725 - RNA, 20 nt, synthetic construct
  source 1..20: mol_type = other RNA
cgcgctggatgccgtcgtgc

SEQ ID NO: 20726 - RNA, 20 nt, synthetic construct
  source 1..20: mol_type = other RNA
ggcatccagcgcgtgctgtt

SEQ ID NO: 20727 - RNA, 20 nt, synthetic construct
  source 1..20: mol_type = other RNA
tgttgccaaacagcacgcgc

SEQ ID NO: 20728 - RNA, 20 nt, synthetic construct
  source 1..20: mol_type = other RNA
ttggcaacaacctgaacttc

SEQ ID NO: 20729 - RNA, 20 nt, synthetic construct
  source 1..20: mol_type = other RNA
gcttgtgcagccagaagttc

SEQ ID NO: 20730 - RNA, 20 nt, synthetic construct
  source 1..20: mol_type = other RNA
gctgcacaagcttgtcttcg

SEQ ID NO: 20731 - RNA, 20 nt, synthetic construct
  source 1..20: mol_type = other RNA
gcttgtcttcgtggatgccg

SEQ ID NO: 20732 - RNA, 20 nt, synthetic construct
  source 1..20: mol_type = other RNA
ggatgccgtggccttcctca

SEQ ID NO: 20733 - RNA, 20 nt, synthetic construct
  source 1..20: mol_type = other RNA
gatgccgtggccttcctcac

SEQ ID NO: 20734 - RNA, 20 nt, synthetic construct
  source 1..20: mol_type = other RNA
atgccgtggccttcctcacg

SEQ ID NO: 20735 - RNA, 20 nt, synthetic construct
  source 1..20: mol_type = other RNA
cttccccgtgaggaaggcca

SEQ ID NO: 20736 - RNA, 20 nt, synthetic construct
  source 1..20: mol_type = other RNA
gaggcgcttccccgtgagga

SEQ ID NO: 20737 - RNA, 20 nt, synthetic construct
  source 1..20: mol_type = other RNA
gggagaggcgcttccccgtg

SEQ ID NO: 20738 - RNA, 20 nt, synthetic construct
  source 1..20: mol_type = other RNA
gaagcgcctctccctgccat

SEQ ID NO: 20739 - RNA, 20 nt, synthetic construct
  source 1..20: mol_type = other RNA
agcggtccaatggcagggag

SEQ ID NO: 20740 - RNA, 20 nt, synthetic construct
  source 1..20: mol_type = other RNA
gccattggaccgctacatcc

SEQ ID NO: 20741 - RNA, 20 nt, synthetic construct
  source 1..20: mol_type = other RNA
gatgtagcggtccaatggca

SEQ ID NO: 20742 - RNA, 20 nt, synthetic construct
  source 1..20: mol_type = other RNA
ggatgtagcggtccaatggc

SEQ ID NO: 20743 - RNA, 20 nt, synthetic construct
  source 1..20: mol_type = other RNA
attggaccgctacatcctgg

SEQ ID NO: 20744 - RNA, 20 nt, synthetic construct
  source 1..20: mol_type = other RNA
accaggatgtagcggtccaa

SEQ ID NO: 20745 - RNA, 20 nt, synthetic construct
  source 1..20: mol_type = other RNA
caatgtccaccaggatgtag

SEQ ID NO: 20746 - RNA, 20 nt, synthetic construct
  source 1..20: mol_type = other RNA
agatgtcatcaatgtccacc

SEQ ID NO: 20747 - RNA, 20 nt, synthetic construct
  source 1..20: mol_type = other RNA
ggacattgatgacatcttcg

SEQ ID NO: 20748 - RNA, 20 nt, synthetic construct
  source 1..20: mol_type = other RNA
gacattgatgacatcttcgt

SEQ ID NO: 20749 - RNA, 20 nt, synthetic construct
  source 1..20: mol_type = other RNA
tgatgacatcttcgtgggca

SEQ ID NO: 20750 - RNA, 20 nt, synthetic construct
  source 1..20: mol_type = other RNA
tgacatcttcgtgggcaagg

SEQ ID NO: 20751 - RNA, 20 nt, synthetic construct
  source 1..20: mol_type = other RNA
gacatcttcgtgggcaagga

SEQ ID NO: 20752 - RNA, 20 nt, synthetic construct
  source 1..20: mol_type = other RNA
caaggagggcacacgcatga

SEQ ID NO: 20753 - RNA, 20 nt, synthetic construct
  source 1..20: mol_type = other RNA
ggagggcacacgcatgaagg

SEQ ID NO: 20754 - RNA, 20 nt, synthetic construct
  source 1..20: mol_type = other RNA
gggcacacgcatgaaggtgg

SEQ ID NO: 20755 - RNA, 20 nt, synthetic construct
  source 1..20: mol_type = other RNA
catgaaggtggaggacgtga

SEQ ID NO: 20756 - RNA, 20 nt, synthetic construct
  source 1..20: mol_type = other RNA
aggtggaggacgtgaaggta

SEQ ID NO: 20757 - RNA, 20 nt, synthetic construct
  source 1..20: mol_type = other RNA
ggaggacgtgaaggtatggc

SEQ ID NO: 20758 - RNA, 20 nt, synthetic construct
  source 1..20: mol_type = other RNA
gaggacgtgaaggtatggcc

SEQ ID NO: 20759 - RNA, 20 nt, synthetic construct
  source 1..20: mol_type = other RNA
aggacgtgaaggtatggccg

SEQ ID NO: 20760 - RNA, 20 nt, synthetic construct
  source 1..20: mol_type = other RNA
ggacgtgaaggtatggccgg

SEQ ID NO: 20761 - RNA, 20 nt, synthetic construct
  source 1..20: mol_type = other RNA
tatggccgggggtgctagac

SEQ ID NO: 20762 - RNA, 20 nt, synthetic construct
  source 1..20: mol_type = other RNA
atggccgggggtgctagacc

SEQ ID NO: 20763 - RNA, 20 nt, synthetic construct
  source 1..20: mol_type = other RNA
cgggggtgctagaccgggca

SEQ ID NO: 20764 - RNA, 20 nt, synthetic construct
  source 1..20: mol_type = other RNA
cttgcccggtctagcacccc

SEQ ID NO: 20765 - RNA, 20 nt, synthetic construct
  source 1..20: mol_type = other RNA
gctagaccgggcaaggcagg

SEQ ID NO: 20766 - RNA, 20 nt, synthetic construct
  source 1..20: mol_type = other RNA
ctagaccgggcaaggcaggt

SEQ ID NO: 20767 - RNA, 20 nt, synthetic construct
  source 1..20: mol_type = other RNA
tagaccgggcaaggcaggtg

SEQ ID NO: 20768 - RNA, 20 nt, synthetic construct
  source 1..20: mol_type = other RNA
cgggcaaggcaggtggggcc

SEQ ID NO: 20769 - RNA, 20 nt, synthetic construct
  source 1..20: mol_type = other RNA
caggccccacctgccttgcc

SEQ ID NO: 20770 - RNA, 20 nt, synthetic construct
  source 1..20: mol_type = other RNA
cctggcaagcttcagccttc

SEQ ID NO: 20771 - RNA, 20 nt, synthetic construct
  source 1..20: mol_type = other RNA
cctgaaggctgaagcttgcc

SEQ ID NO: 20772 - RNA, 20 nt, synthetic construct
  source 1..20: mol_type = other RNA
agccttcaggtgccccatcg

SEQ ID NO: 20773 - RNA, 20 nt, synthetic construct
  source 1..20: mol_type = other RNA
gccttcaggtgccccatcgt

SEQ ID NO: 20774 - RNA, 20 nt, synthetic construct
  source 1..20: mol_type = other RNA
acccacgatggggcacctga

SEQ ID NO: 20775 - RNA, 20 nt, synthetic construct
  source 1..20: mol_type = other RNA
gacagggcacacccacgatg

SEQ ID NO: 20776 - RNA, 20 nt, synthetic construct
  source 1..20: mol_type = other RNA
agacagggcacacccacgat

SEQ ID NO: 20777 - RNA, 20 nt, synthetic construct
  source 1..20: mol_type = other RNA
cagacagggcacacccacga

SEQ ID NO: 20778 - RNA, 20 nt, synthetic construct
  source 1..20: mol_type = other RNA
tgtctgcatctcccctatgc

SEQ ID NO: 20779 - RNA, 20 nt, synthetic construct
  source 1..20: mol_type = other RNA
gtctgcatctcccctatgct

SEQ ID NO: 20780 - RNA, 20 nt, synthetic construct
  source 1..20: mol_type = other RNA
gcataggggagatgcagaca

SEQ ID NO: 20781 - RNA, 20 nt, synthetic construct
  source 1..20: mol_type = other RNA
agcataggggagatgcagac

SEQ ID NO: 20782 - RNA, 20 nt, synthetic construct
  source 1..20: mol_type = other RNA
ttaagtaactcccagcatag

SEQ ID NO: 20783 - RNA, 20 nt, synthetic construct
  source 1..20: mol_type = other RNA
tttaagtaactcccagcata

SEQ ID NO: 20784 - RNA, 20 nt, synthetic construct
  source 1..20: mol_type = other RNA
ttttaagtaactcccagcat

SEQ ID NO: 20785 - RNA, 20 nt, synthetic construct
  source 1..20: mol_type = other RNA
attataaagaatgtcaagga

SEQ ID NO: 20786 - RNA, 20 nt, synthetic construct
  source 1..20: mol_type = other RNA
aaaaattataaagaatgtca

SEQ ID NO: 20787 - RNA, 20 nt, synthetic construct
  source 1..20: mol_type = other RNA
ttctttataatttttgaaca

SEQ ID NO: 20788 - RNA, 20 nt, synthetic construct
  source 1..20: mol_type = other RNA
tctttataatttttgaacaa

SEQ ID NO: 20789 - RNA, 20 nt, synthetic construct
  source 1..20: mol_type = other RNA
cgttttttcactgccctcag

SEQ ID NO: 20790 - RNA, 20 nt, synthetic construct
  source 1..20: mol_type = other RNA
gttttttcactgccctcagt

SEQ ID NO: 20791 - RNA, 20 nt, synthetic construct
  source 1..20: mol_type = other RNA
ctgagggcagtgaaaaaacg

SEQ ID NO: 20792 - RNA, 20 nt, synthetic construct
  source 1..20: mol_type = other RNA
ctgccctcagtgggaaaagc

SEQ ID NO: 20793 - RNA, 20 nt, synthetic construct
  source 1..20: mol_type = other RNA
tgccctcagtgggaaaagca

SEQ ID NO: 20794 - RNA, 20 nt, synthetic construct
  source 1..20: mol_type = other RNA
ctccctgcttttcccactga

SEQ ID NO: 20795 - RNA, 20 nt, synthetic construct
  source 1..20: mol_type = other RNA
gctccctgcttttcccactg

SEQ ID NO: 20796 - RNA, 20 nt, synthetic construct
  source 1..20: mol_type = other RNA
tgggaaaagcagggagctcc

SEQ ID NO: 20797 - RNA, 20 nt, synthetic construct
  source 1..20: mol_type = other RNA
ggaatgagtgagggaaagcc

SEQ ID NO: 20798 - RNA, 20 nt, synthetic construct
  source 1..20: mol_type = other RNA
ggggagaaaggaatgagtga

SEQ ID NO: 20799 - RNA, 20 nt, synthetic construct
  source 1..20: mol_type = other RNA
aggggagaaaggaatgagtg

SEQ ID NO: 20800 - RNA, 20 nt, synthetic construct
  source 1..20: mol_type = other RNA
ctttctcccctgcctgtcct

SEQ ID NO: 20801 - RNA, 20 nt, synthetic construct
  source 1..20: mol_type = other RNA
ctaggacaggcaggggagaa

SEQ ID NO: 20802 - RNA, 20 nt, synthetic construct
  source 1..20: mol_type = other RNA
acagggcctaggacaggcag

SEQ ID NO: 20803 - RNA, 20 nt, synthetic construct
  source 1..20: mol_type = other RNA
aacagggcctaggacaggca

SEQ ID NO: 20804 - RNA, 20 nt, synthetic construct
  source 1..20: mol_type = other RNA
aaacagggcctaggacaggc

SEQ ID NO: 20805 - RNA, 20 nt, synthetic construct
  source 1..20: mol_type = other RNA
tgtcaaacagggcctaggac

SEQ ID NO: 20806 - RNA, 20 nt, synthetic construct
  source 1..20: mol_type = other RNA
ctgtgtgtcaaacagggcct

SEQ ID NO: 20807 - RNA, 20 nt, synthetic construct
  source 1..20: mol_type = other RNA
ttcgttctgtgtgtcaaaca

SEQ ID NO: 20808 - RNA, 20 nt, synthetic construct
  source 1..20: mol_type = other RNA
gttcgttctgtgtgtcaaac

SEQ ID NO: 20809 - RNA, 20 nt, synthetic construct
  source 1..20: mol_type = other RNA
cccaaacttcaccttcaacc

SEQ ID NO: 20810 - RNA, 20 nt, synthetic construct
  source 1..20: mol_type = other RNA
ccaaacttcaccttcaacct

SEQ ID NO: 20811 - RNA, 20 nt, synthetic construct
  source 1..20: mol_type = other RNA
ccaggttgaaggtgaagttt

SEQ ID NO: 20812 - RNA, 20 nt, synthetic construct
  source 1..20: mol_type = other RNA
cccaggttgaaggtgaagtt

SEQ ID NO: 20813 - RNA, 20 nt, synthetic construct
  source 1..20: mol_type = other RNA
accttcaacctgggctactc

SEQ ID NO: 20814 - RNA, 20 nt, synthetic construct
  source 1..20: mol_type = other RNA
ccttcaacctgggctactca

SEQ ID NO: 20815 - RNA, 20 nt, synthetic construct
  source 1..20: mol_type = other RNA
ccctgagtagcccaggttga

SEQ ID NO: 20816 - RNA, 20 nt, synthetic construct
  source 1..20: mol_type = other RNA
agaatttccctgagtagccc

SEQ ID NO: 20817 - RNA, 20 nt, synthetic construct
  source 1..20: mol_type = other RNA
tcagggaaattcttccacac

SEQ ID NO: 20818 - RNA, 20 nt, synthetic construct
  source 1..20: mol_type = other RNA
aattcttccacacaggtaag

SEQ ID NO: 20819 - RNA, 20 nt, synthetic construct
  source 1..20: mol_type = other RNA
attcttccacacaggtaagt

SEQ ID NO: 20820 - RNA, 20 nt, synthetic construct
  source 1..20: mol_type = other RNA
ggcaggcccacttacctgtg

SEQ ID NO: 20821 - RNA, 20 nt, synthetic construct
  source 1..20: mol_type = other RNA
ttgctagtgagggcaggggc

SEQ ID NO: 20822 - RNA, 20 nt, synthetic construct
  source 1..20: mol_type = other RNA
tgccctcactagcaacttcc

SEQ ID NO: 20823 - RNA, 20 nt, synthetic construct
  source 1..20: mol_type = other RNA
gaagttgctagtgagggcag

SEQ ID NO: 20824 - RNA, 20 nt, synthetic construct
  source 1..20: mol_type = other RNA
ggaagttgctagtgagggca

SEQ ID NO: 20825 - RNA, 20 nt, synthetic construct
  source 1..20: mol_type = other RNA
tggaagttgctagtgagggc

SEQ ID NO: 20826 - RNA, 20 nt, synthetic construct
  source 1..20: mol_type = other RNA
gtcctggaagttgctagtga

SEQ ID NO: 20827 - RNA, 20 nt, synthetic construct
  source 1..20: mol_type = other RNA
agtcctggaagttgctagtg

SEQ ID NO: 20828 - RNA, 20 nt, synthetic construct
  source 1..20: mol_type = other RNA
gtttgggtgctgaggagtcc

SEQ ID NO: 20829 - RNA, 20 nt, synthetic construct
  source 1..20: mol_type = other RNA
ctttgagggtttgggtgctg

SEQ ID NO: 20830 - RNA, 20 nt, synthetic construct
  source 1..20: mol_type = other RNA
gatgggtgctttgagggttt

SEQ ID NO: 20831 - RNA, 20 nt, synthetic construct
  source 1..20: mol_type = other RNA
ggatgggtgctttgagggtt

SEQ ID NO: 20832 - RNA, 20 nt, synthetic construct
  source 1..20: mol_type = other RNA
cctcaaagcacccatccatg

SEQ ID NO: 20833 - RNA, 20 nt, synthetic construct
  source 1..20: mol_type = other RNA
ctcaaagcacccatccatga

SEQ ID NO: 20834 - RNA, 20 nt, synthetic construct
  source 1..20: mol_type = other RNA
ctcatggatgggtgctttga

SEQ ID NO: 20835 - RNA, 20 nt, synthetic construct
  source 1..20: mol_type = other RNA
cctcatggatgggtgctttg

SEQ ID NO: 20836 - RNA, 20 nt, synthetic construct
  source 1..20: mol_type = other RNA
gcacccatccatgagggcag

SEQ ID NO: 20837 - RNA, 20 nt, synthetic construct
  source 1..20: mol_type = other RNA
cacccatccatgagggcagc

SEQ ID NO: 20838 - RNA, 20 nt, synthetic construct
  source 1..20: mol_type = other RNA
ccatccatgagggcagcggg

SEQ ID NO: 20839 - RNA, 20 nt, synthetic construct
  source 1..20: mol_type = other RNA
catccatgagggcagcgggt

SEQ ID NO: 20840 - RNA, 20 nt, synthetic construct
  source 1..20: mol_type = other RNA
cacccgctgccctcatggat

SEQ ID NO: 20841 - RNA, 20 nt, synthetic construct
  source 1..20: mol_type = other RNA
ccacccgctgccctcatgga

SEQ ID NO: 20842 - RNA, 20 nt, synthetic construct
  source 1..20: mol_type = other RNA
agggcagcgggtgggtttac

SEQ ID NO: 20843 - RNA, 20 nt, synthetic construct
  source 1..20: mol_type = other RNA
ggtttactggcccacattag

SEQ ID NO: 20844 - RNA, 20 nt, synthetic construct
  source 1..20: mol_type = other RNA
ctggcccacattagaggcag

SEQ ID NO: 20845 - RNA, 20 nt, synthetic construct
  source 1..20: mol_type = other RNA
gctgcctggaagagttatct

SEQ ID NO: 20846 - RNA, 20 nt, synthetic construct
  source 1..20: mol_type = other RNA
agctgcctggaagagttatc

SEQ ID NO: 20847 - RNA, 20 nt, synthetic construct
  source 1..20: mol_type = other RNA
aactcttccaggcagctcct

SEQ ID NO: 20848 - RNA, 20 nt, synthetic construct
  source 1..20: mol_type = other RNA
tcttccaggcagctcctggg

SEQ ID NO: 20849 - RNA, 20 nt, synthetic construct
  source 1..20: mol_type = other RNA
cttccaggcagctcctgggt

SEQ ID NO: 20850 - RNA, 20 nt, synthetic construct
  source 1..20: mol_type = other RNA
ggcagctcctgggtgggctc

SEQ ID NO: 20851 - RNA, 20 nt, synthetic construct
  source 1..20: mol_type = other RNA
gagcccacccaggagctgcc

SEQ ID NO: 20852 - RNA, 20 nt, synthetic construct
  source 1..20: mol_type = other RNA
agcatggccagagcccaccc

SEQ ID NO: 20853 - RNA, 20 nt, synthetic construct
  source 1..20: mol_type = other RNA
ggccatgctctcccatcccc

SEQ ID NO: 20854 - RNA, 20 nt, synthetic construct
  source 1..20: mol_type = other RNA
gctctcccatccccaggcac

SEQ ID NO: 20855 - RNA, 20 nt, synthetic construct
  source 1..20: mol_type = other RNA
tgcctggggatgggagagca

SEQ ID NO: 20856 - RNA, 20 nt, synthetic construct
  source 1..20: mol_type = other RNA
ccatccccaggcacaggccc

SEQ ID NO: 20857 - RNA, 20 nt, synthetic construct
  source 1..20: mol_type = other RNA
ctgggcctgtgcctggggat

SEQ ID NO: 20858 - RNA, 20 nt, synthetic construct
  source 1..20: mol_type = other RNA
cctgggcctgtgcctgggga

SEQ ID NO: 20859 - RNA, 20 nt, synthetic construct
  source 1..20: mol_type = other RNA
caggcacaggcccaggttag

SEQ ID NO: 20860 - RNA, 20 nt, synthetic construct
  source 1..20: mol_type = other RNA
aggcacaggcccaggttaga

SEQ ID NO: 20861 - RNA, 20 nt, synthetic construct
  source 1..20: mol_type = other RNA
ctaacctgggcctgtgcctg

SEQ ID NO: 20862 - RNA, 20 nt, synthetic construct
  source 1..20: mol_type = other RNA
tctaacctgggcctgtgcct

SEQ ID NO: 20863 - RNA, 20 nt, synthetic construct
  source 1..20: mol_type = other RNA
ctctaacctgggcctgtgcc

SEQ ID NO: 20864 - RNA, 20 nt, synthetic construct
  source 1..20: mol_type = other RNA
gcccaggttagagggcctca

SEQ ID NO: 20865 - RNA, 20 nt, synthetic construct
  source 1..20: mol_type = other RNA
gccatgaggccctctaacct

SEQ ID NO: 20866 - RNA, 20 nt, synthetic construct
  source 1..20: mol_type = other RNA
ggccatgaggccctctaacc

SEQ ID NO: 20867 - RNA, 20 nt, synthetic construct
  source 1..20: mol_type = other RNA
tagagggcctcatggcccag

SEQ ID NO: 20868 - RNA, 20 nt, synthetic construct
  source 1..20: mol_type = other RNA
agagggcctcatggcccagt

SEQ ID NO: 20869 - RNA, 20 nt, synthetic construct
  source 1..20: mol_type = other RNA
gggcctcatggcccagtggg

SEQ ID NO: 20870 - RNA, 20 nt, synthetic construct
  source 1..20: mol_type = other RNA
gaaccacccactgggccatg

SEQ ID NO: 20871 - RNA, 20 nt, synthetic construct
  source 1..20: mol_type = other RNA
gcagctcagaaccacccact

SEQ ID NO: 20872 - RNA, 20 nt, synthetic construct
  source 1..20: mol_type = other RNA
ggcagctcagaaccacccac

SEQ ID NO: 20873 - RNA, 20 nt, synthetic construct
  source 1..20: mol_type = other RNA
tgagctgcctgtgttgctgc

SEQ ID NO: 20874 - RNA, 20 nt, synthetic construct
  source 1..20: mol_type = other RNA
attggtacctgcagcaacac

SEQ ID NO: 20875 - RNA, 20 nt, synthetic construct
  source 1..20: mol_type = other RNA
tgctgcaggtaccaatgctg

SEQ ID NO: 20876 - RNA, 20 nt, synthetic construct
  source 1..20: mol_type = other RNA
ggtaccaatgctgaggacgc

SEQ ID NO: 20877 - RNA, 20 nt, synthetic construct
  source 1..20: mol_type = other RNA
gtaccaatgctgaggacgct

SEQ ID NO: 20878 - RNA, 20 nt, synthetic construct
  source 1..20: mol_type = other RNA
taccaatgctgaggacgctg

SEQ ID NO: 20879 - RNA, 20 nt, synthetic construct
  source 1..20: mol_type = other RNA
atccccagcgtcctcagcat

SEQ ID NO: 20880 - RNA, 20 nt, synthetic construct
  source 1..20: mol_type = other RNA
tctgctgctgtcgtatgtga

SEQ ID NO: 20881 - RNA, 20 nt, synthetic construct
  source 1..20: mol_type = other RNA
tgtcgtatgtgaaggagttc

SEQ ID NO: 20882 - RNA, 20 nt, synthetic construct
  source 1..20: mol_type = other RNA
cgtatgtgaaggagttctgg

SEQ ID NO: 20883 - RNA, 20 nt, synthetic construct
  source 1..20: mol_type = other RNA
tctggtggttcccccacatg

SEQ ID NO: 20884 - RNA, 20 nt, synthetic construct
  source 1..20: mol_type = other RNA
gcatgtggctccacatgtgg

SEQ ID NO: 20885 - RNA, 20 nt, synthetic construct
  source 1..20: mol_type = other RNA
tgcatgtggctccacatgtg

SEQ ID NO: 20886 - RNA, 20 nt, synthetic construct
  source 1..20: mol_type = other RNA
ctgcatgtggctccacatgt

SEQ ID NO: 20887 - RNA, 20 nt, synthetic construct
  source 1..20: mol_type = other RNA
gctgcatgtggctccacatg

SEQ ID NO: 20888 - RNA, 20 nt, synthetic construct
  source 1..20: mol_type = other RNA
ggaaaaggtggggctgcatg

SEQ ID NO: 20889 - RNA, 20 nt, synthetic construct
  source 1..20: mol_type = other RNA
gactggttgtggaaaaggtg

SEQ ID NO: 20890 - RNA, 20 nt, synthetic construct
  source 1..20: mol_type = other RNA
ggactggttgtggaaaaggt

SEQ ID NO: 20891 - RNA, 20 nt, synthetic construct
  source 1..20: mol_type = other RNA
cggactggttgtggaaaagg

SEQ ID NO: 20892 - RNA, 20 nt, synthetic construct
  source 1..20: mol_type = other RNA
tttccacaaccagtccgtgt

SEQ ID NO: 20893 - RNA, 20 nt, synthetic construct
  source 1..20: mol_type = other RNA
acacggactggttgtggaaa

SEQ ID NO: 20894 - RNA, 20 nt, synthetic construct
  source 1..20: mol_type = other RNA
cggccaacacggactggttg

SEQ ID NO: 20895 - RNA, 20 nt, synthetic construct
  source 1..20: mol_type = other RNA
gtccgtgttggccgagcaga

SEQ ID NO: 20896 - RNA, 20 nt, synthetic construct
  source 1..20: mol_type = other RNA
tctgctcggccaacacggac

SEQ ID NO: 20897 - RNA, 20 nt, synthetic construct
  source 1..20: mol_type = other RNA
ggccatctgctcggccaaca

SEQ ID NO: 20898 - RNA, 20 nt, synthetic construct
  source 1..20: mol_type = other RNA
cttgttcaaggccatctgct

SEQ ID NO: 20899 - RNA, 20 nt, synthetic construct
  source 1..20: mol_type = other RNA
gacagcgaacttcttgttca

SEQ ID NO: 20900 - RNA, 20 nt, synthetic construct
  source 1..20: mol_type = other RNA
tcgtgagtaagattccttgc

SEQ ID NO: 20901 - RNA, 20 nt, synthetic construct
  source 1..20: mol_type = other RNA
cgtgagtaagattccttgca

SEQ ID NO: 20902 - RNA, 20 nt, synthetic construct
  source 1..20: mol_type = other RNA
agattccttgcagggcagag

SEQ ID NO: 20903 - RNA, 20 nt, synthetic construct
  source 1..20: mol_type = other RNA
gattccttgcagggcagagc

SEQ ID NO: 20904 - RNA, 20 nt, synthetic construct
  source 1..20: mol_type = other RNA
attccttgcagggcagagcg

SEQ ID NO: 20905 - RNA, 20 nt, synthetic construct
  source 1..20: mol_type = other RNA
ccttgcagggcagagcgggg

SEQ ID NO: 20906 - RNA, 20 nt, synthetic construct
  source 1..20: mol_type = other RNA
cttgcagggcagagcggggc

SEQ ID NO: 20907 - RNA, 20 nt, synthetic construct
  source 1..20: mol_type = other RNA
ccgccccgctctgccctgca

SEQ ID NO: 20908 - RNA, 20 nt, synthetic construct
  source 1..20: mol_type = other RNA
gggcagagcggggcgggcta

SEQ ID NO: 20909 - RNA, 20 nt, synthetic construct
  source 1..20: mol_type = other RNA
ggcagagcggggcgggctaa

SEQ ID NO: 20910 - RNA, 20 nt, synthetic construct
  source 1..20: mol_type = other RNA
gagcggggcgggctaagggc

SEQ ID NO: 20911 - RNA, 20 nt, synthetic construct
  source 1..20: mol_type = other RNA
agcggggcgggctaagggct

SEQ ID NO: 20912 - RNA, 20 nt, synthetic construct
  source 1..20: mol_type = other RNA
gggcgggctaagggctgggc

SEQ ID NO: 20913 - RNA, 20 nt, synthetic construct
  source 1..20: mol_type = other RNA
cgggctaagggctgggctgg

SEQ ID NO: 20914 - RNA, 20 nt, synthetic construct
  source 1..20: mol_type = other RNA
gggctggaggtccagactgc

SEQ ID NO: 20915 - RNA, 20 nt, synthetic construct
  source 1..20: mol_type = other RNA
gcagcaagaggccagcagtc

SEQ ID NO: 20916 - RNA, 20 nt, synthetic construct
  source 1..20: mol_type = other RNA
cagactgcaaaagcagcaag

SEQ ID NO: 20917 - RNA, 20 nt, synthetic construct
  source 1..20: mol_type = other RNA
gcttttgcagtctgctctga

SEQ ID NO: 20918 - RNA, 20 nt, synthetic construct
  source 1..20: mol_type = other RNA
cggatttttactaacacctc

SEQ ID NO: 20919 - RNA, 20 nt, synthetic construct
  source 1..20: mol_type = other RNA
ggatttttactaacacctct

SEQ ID NO: 20920 - RNA, 20 nt, synthetic construct
  source 1..20: mol_type = other RNA
tttactaacacctctgggcc

SEQ ID NO: 20921 - RNA, 20 nt, synthetic construct
  source 1..20: mol_type = other RNA
ttactaacacctctgggcca

SEQ ID NO: 20922 - RNA, 20 nt, synthetic construct
  source 1..20: mol_type = other RNA
ggttaggtcggcatggctgc

SEQ ID NO: 20923 - RNA, 20 nt, synthetic construct
  source 1..20: mol_type = other RNA
aatcagaggttaggtcggca

SEQ ID NO: 20924 - RNA, 20 nt, synthetic construct
  source 1..20: mol_type = other RNA
agagaaatcagaggttaggt

SEQ ID NO: 20925 - RNA, 20 nt, synthetic construct
  source 1..20: mol_type = other RNA
ggagagagaaatcagaggtt

SEQ ID NO: 20926 - RNA, 20 nt, synthetic construct
  source 1..20: mol_type = other RNA
gaatgggagagagaaatcag

SEQ ID NO: 20927 - RNA, 20 nt, synthetic construct
  source 1..20: mol_type = other RNA
ttctctctcccattctacaa

SEQ ID NO: 20928 - RNA, 20 nt, synthetic construct
  source 1..20: mol_type = other RNA
tctctctcccattctacaaa

SEQ ID NO: 20929 - RNA, 20 nt, synthetic construct
  source 1..20: mol_type = other RNA
ctctctcccattctacaaag

SEQ ID NO: 20930 - RNA, 20 nt, synthetic construct
  source 1..20: mol_type = other RNA
tctctcccattctacaaagg

SEQ ID NO: 20931 - RNA, 20 nt, synthetic construct
  source 1..20: mol_type = other RNA
ctctcccattctacaaaggg

SEQ ID NO: 20932 - RNA, 20 nt, synthetic construct
  source 1..20: mol_type = other RNA
cattctacaaaggggggata

SEQ ID NO: 20933 - RNA, 20 nt, synthetic construct
  source 1..20: mol_type = other RNA
ttatcccccctttgtagaat

SEQ ID NO: 20934 - RNA, 20 nt, synthetic construct
  source 1..20: mol_type = other RNA
cttatcccccctttgtagaa

SEQ ID NO: 20935 - RNA, 20 nt, synthetic construct
  source 1..20: mol_type = other RNA
aaaggggggataaggcccaa

SEQ ID NO: 20936 - RNA, 20 nt, synthetic construct
  source 1..20: mol_type = other RNA
aaggggggataaggcccaaa

SEQ ID NO: 20937 - RNA, 20 nt, synthetic construct
  source 1..20: mol_type = other RNA
aggggggataaggcccaaag

SEQ ID NO: 20938 - RNA, 20 nt, synthetic construct
  source 1..20: mol_type = other RNA
gggataaggcccaaagggga

SEQ ID NO: 20939 - RNA, 20 nt, synthetic construct
  source 1..20: mol_type = other RNA
cataggggtccttccccttt

SEQ ID NO: 20940 - RNA, 20 nt, synthetic construct
  source 1..20: mol_type = other RNA
gcataggggtccttcccctt

SEQ ID NO: 20941 - RNA, 20 nt, synthetic construct
  source 1..20: mol_type = other RNA
aaggacccctatgctcaccc

SEQ ID NO: 20942 - RNA, 20 nt, synthetic construct
  source 1..20: mol_type = other RNA
cccctatgctcaccctggcc

SEQ ID NO: 20943 - RNA, 20 nt, synthetic construct
  source 1..20: mol_type = other RNA
ccaggccagggtgagcatag

SEQ ID NO: 20944 - RNA, 20 nt, synthetic construct
  source 1..20: mol_type = other RNA
accaggccagggtgagcata

SEQ ID NO: 20945 - RNA, 20 nt, synthetic construct
  source 1..20: mol_type = other RNA
gaccaggccagggtgagcat

SEQ ID NO: 20946 - RNA, 20 nt, synthetic construct
  source 1..20: mol_type = other RNA
ggcctggtcatcctctccct

SEQ ID NO: 20947 - RNA, 20 nt, synthetic construct
  source 1..20: mol_type = other RNA
gggagaggatgaccaggcca

SEQ ID NO: 20948 - RNA, 20 nt, synthetic construct
  source 1..20: mol_type = other RNA
agggagaggatgaccaggcc

SEQ ID NO: 20949 - RNA, 20 nt, synthetic construct
  source 1..20: mol_type = other RNA
tcatcctctccctaggagca

SEQ ID NO: 20950 - RNA, 20 nt, synthetic construct
  source 1..20: mol_type = other RNA
aatgccatgctcctagggag

SEQ ID NO: 20951 - RNA, 20 nt, synthetic construct
  source 1..20: mol_type = other RNA
gtgggaatgccatgctccta

SEQ ID NO: 20952 - RNA, 20 nt, synthetic construct
  source 1..20: mol_type = other RNA
tgtgggaatgccatgctcct

SEQ ID NO: 20953 - RNA, 20 nt, synthetic construct
  source 1..20: mol_type = other RNA
gcatggcattcccacagaca

SEQ ID NO: 20954 - RNA, 20 nt, synthetic construct
  source 1..20: mol_type = other RNA
catggcattcccacagacat

SEQ ID NO: 20955 - RNA, 20 nt, synthetic construct
  source 1..20: mol_type = other RNA
atggcattcccacagacatg

SEQ ID NO: 20956 - RNA, 20 nt, synthetic construct
  source 1..20: mol_type = other RNA
cacagacatggggtatgcag

SEQ ID NO: 20957 - RNA, 20 nt, synthetic construct
  source 1..20: mol_type = other RNA
actgcataccccatgtctgt

SEQ ID NO: 20958 - RNA, 20 nt, synthetic construct
  source 1..20: mol_type = other RNA
cactgcataccccatgtctg

SEQ ID NO: 20959 - RNA, 20 nt, synthetic construct
  source 1..20: mol_type = other RNA
tgcagtggcgccccaccact

SEQ ID NO: 20960 - RNA, 20 nt, synthetic construct
  source 1..20: mol_type = other RNA
gcagtggcgccccaccactc

SEQ ID NO: 20961 - RNA, 20 nt, synthetic construct
  source 1..20: mol_type = other RNA
gggtacacgcccgagtggtg

SEQ ID NO: 20962 - RNA, 20 nt, synthetic construct
  source 1..20: mol_type = other RNA
ggggtacacgcccgagtggt

SEQ ID NO: 20963 - RNA, 20 nt, synthetic construct
  source 1..20: mol_type = other RNA
cggggtacacgcccgagtgg

SEQ ID NO: 20964 - RNA, 20 nt, synthetic construct
  source 1..20: mol_type = other RNA
gcacggggtacacgcccgag

SEQ ID NO: 20965 - RNA, 20 nt, synthetic construct
  source 1..20: mol_type = other RNA
cgtgcacgtgcagctgtacg

SEQ ID NO: 20966 - RNA, 20 nt, synthetic construct
  source 1..20: mol_type = other RNA
cgtacagctgcacgtgcacg

SEQ ID NO: 20967 - RNA, 20 nt, synthetic construct
  source 1..20: mol_type = other RNA
tcgtacagctgcacgtgcac

SEQ ID NO: 20968 - RNA, 20 nt, synthetic construct
  source 1..20: mol_type = other RNA
ctcgtacagctgcacgtgca

SEQ ID NO: 20969 - RNA, 20 nt, synthetic construct
  source 1..20: mol_type = other RNA
acgtgcagctgtacgaggct

SEQ ID NO: 20970 - RNA, 20 nt, synthetic construct
  source 1..20: mol_type = other RNA
gctgtacgaggcttggaagc

SEQ ID NO: 20971 - RNA, 20 nt, synthetic construct
  source 1..20: mol_type = other RNA
acgaggcttggaagcaggtg

SEQ ID NO: 20972 - RNA, 20 nt, synthetic construct
  source 1..20: mol_type = other RNA
gagcatccgcgtgaccagca

SEQ ID NO: 20973 - RNA, 20 nt, synthetic construct
  source 1..20: mol_type = other RNA
catccgcgtgaccagcacgg

SEQ ID NO: 20974 - RNA, 20 nt, synthetic construct
  source 1..20: mol_type = other RNA
actcctccgtgctggtcacg

SEQ ID NO: 20975 - RNA, 20 nt, synthetic construct
  source 1..20: mol_type = other RNA
gtgggggtactcctccgtgc

SEQ ID NO: 20976 - RNA, 20 nt, synthetic construct
  source 1..20: mol_type = other RNA
agcgggctggcttcaggtgg

SEQ ID NO: 20977 - RNA, 20 nt, synthetic construct
  source 1..20: mol_type = other RNA
tagcgggctggcttcaggtg

SEQ ID NO: 20978 - RNA, 20 nt, synthetic construct
  source 1..20: mol_type = other RNA
gtagcgggctggcttcaggt

SEQ ID NO: 20979 - RNA, 20 nt, synthetic construct
  source 1..20: mol_type = other RNA
ggtagcgggctggcttcagg

SEQ ID NO: 20980 - RNA, 20 nt, synthetic construct
  source 1..20: mol_type = other RNA
aagccagcccgctaccgccg

SEQ ID NO: 20981 - RNA, 20 nt, synthetic construct
  source 1..20: mol_type = other RNA
ggcggtagcgggctggcttc

SEQ ID NO: 20982 - RNA, 20 nt, synthetic construct
  source 1..20: mol_type = other RNA
aagccacggcggtagcgggc

SEQ ID NO: 20983 - RNA, 20 nt, synthetic construct
  source 1..20: mol_type = other RNA
gatgaagccacggcggtagc

SEQ ID NO: 20984 - RNA, 20 nt, synthetic construct
  source 1..20: mol_type = other RNA
ggatgaagccacggcggtag

SEQ ID NO: 20985 - RNA, 20 nt, synthetic construct
  source 1..20: mol_type = other RNA
cgccgtggcttcatccacaa

SEQ ID NO: 20986 - RNA, 20 nt, synthetic construct
  source 1..20: mol_type = other RNA
cattgtggatgaagccacgg

SEQ ID NO: 20987 - RNA, 20 nt, synthetic construct
  source 1..20: mol_type = other RNA
tgccattgtggatgaagcca

SEQ ID NO: 20988 - RNA, 20 nt, synthetic construct
  source 1..20: mol_type = other RNA
cttcatccacaatggcatca

SEQ ID NO: 20989 - RNA, 20 nt, synthetic construct
  source 1..20: mol_type = other RNA
cacaatggcatcatggtgag

SEQ ID NO: 20990 - RNA, 20 nt, synthetic construct
  source 1..20: mol_type = other RNA
acaatggcatcatggtgagt

SEQ ID NO: 20991 - RNA, 20 nt, synthetic construct
  source 1..20: mol_type = other RNA
cactcaccatgatgccattg

SEQ ID NO: 20992 - RNA, 20 nt, synthetic construct
  source 1..20: mol_type = other RNA
catcatggtgagtgggcccc

SEQ ID NO: 20993 - RNA, 20 nt, synthetic construct
  source 1..20: mol_type = other RNA
gagtgggcccctggaagccc

SEQ ID NO: 20994 - RNA, 20 nt, synthetic construct
  source 1..20: mol_type = other RNA
tgggcccctggaagcccagg

SEQ ID NO: 20995 - RNA, 20 nt, synthetic construct
  source 1..20: mol_type = other RNA
gcccctggaagcccaggagg

SEQ ID NO: 20996 - RNA, 20 nt, synthetic construct
  source 1..20: mol_type = other RNA
cccctggaagcccaggaggt

SEQ ID NO: 20997 - RNA, 20 nt, synthetic construct
  source 1..20: mol_type = other RNA
cccacctcctgggcttccag

SEQ ID NO: 20998 - RNA, 20 nt, synthetic construct
  source 1..20: mol_type = other RNA
tcccacctcctgggcttcca

SEQ ID NO: 20999 - RNA, 20 nt, synthetic construct
  source 1..20: mol_type = other RNA
ctcccacctcctgggcttcc

SEQ ID NO: 21000 - RNA, 20 nt, synthetic construct
  source 1..20: mol_type = other RNA
tctccattctcccacctcct

SEQ ID NO: 21001 - RNA, 20 nt, synthetic construct
  source 1..20: mol_type = other RNA
ctctccattctcccacctcc

SEQ ID NO: 21002 - RNA, 20 nt, synthetic construct
  source 1..20: mol_type = other RNA
tgtgtgtgcatacgctgtcc

SEQ ID NO: 21003 - RNA, 20 nt, synthetic construct
  source 1..20: mol_type = other RNA
atacgctgtcctggtaagca

SEQ ID NO: 21004 - RNA, 20 nt, synthetic construct
  source 1..20: mol_type = other RNA
tgtcctggtaagcacggctc

SEQ ID NO: 21005 - RNA, 20 nt, synthetic construct
  source 1..20: mol_type = other RNA
taagcacggctctggtttgc

SEQ ID NO: 21006 - RNA, 20 nt, synthetic construct
  source 1..20: mol_type = other RNA
cggctctggtttgctggctt

SEQ ID NO: 21007 - RNA, 20 nt, synthetic construct
  source 1..20: mol_type = other RNA
ggctctggtttgctggctta

SEQ ID NO: 21008 - RNA, 20 nt, synthetic construct
  source 1..20: mol_type = other RNA
gctctggtttgctggcttag

SEQ ID NO: 21009 - RNA, 20 nt, synthetic construct
  source 1..20: mol_type = other RNA
acatggagactgcctttctg

SEQ ID NO: 21010 - RNA, 20 nt, synthetic construct
  source 1..20: mol_type = other RNA
tcagaaaggcagtctccatg

SEQ ID NO: 21011 - RNA, 20 nt, synthetic construct
  source 1..20: mol_type = other RNA
ctgcctttctgaggagcagc

SEQ ID NO: 21012 - RNA, 20 nt, synthetic construct
  source 1..20: mol_type = other RNA
tgcctttctgaggagcagct

SEQ ID NO: 21013 - RNA, 20 nt, synthetic construct
  source 1..20: mol_type = other RNA
ggcccagctgctcctcagaa

SEQ ID NO: 21014 - RNA, 20 nt, synthetic construct
  source 1..20: mol_type = other RNA
agctgggccttcttcctctg

SEQ ID NO: 21015 - RNA, 20 nt, synthetic construct
  source 1..20: mol_type = other RNA
gactcttcctcagaggaaga

SEQ ID NO: 21016 - RNA, 20 nt, synthetic construct
  source 1..20: mol_type = other RNA
gtgggaggactcttcctcag

SEQ ID NO: 21017 - RNA, 20 nt, synthetic construct
  source 1..20: mol_type = other RNA
cccaccaccctcatgccaga

SEQ ID NO: 21018 - RNA, 20 nt, synthetic construct
  source 1..20: mol_type = other RNA
tctggcatgagggtggtggg

SEQ ID NO: 21019 - RNA, 20 nt, synthetic construct
  source 1..20: mol_type = other RNA
ccttctggcatgagggtggt

SEQ ID NO: 21020 - RNA, 20 nt, synthetic construct
  source 1..20: mol_type = other RNA
gccttctggcatgagggtgg

SEQ ID NO: 21021 - RNA, 20 nt, synthetic construct
  source 1..20: mol_type = other RNA
ggtgccttctggcatgaggg

SEQ ID NO: 21022 - RNA, 20 nt, synthetic construct
  source 1..20: mol_type = other RNA
tatggtgccttctggcatga

SEQ ID NO: 21023 - RNA, 20 nt, synthetic construct
  source 1..20: mol_type = other RNA
ctatggtgccttctggcatg

SEQ ID NO: 21024 - RNA, 20 nt, synthetic construct
  source 1..20: mol_type = other RNA
agaggagctatggtgccttc

SEQ ID NO: 21025 - RNA, 20 nt, synthetic construct
  source 1..20: mol_type = other RNA
ggggtgggggagaggagcta

SEQ ID NO: 21026 - RNA, 20 nt, synthetic construct
  source 1..20: mol_type = other RNA
ctctcccccaccccctcctc

SEQ ID NO: 21027 - RNA, 20 nt, synthetic construct
  source 1..20: mol_type = other RNA
ctgaggagggggtgggggag

SEQ ID NO: 21028 - RNA, 20 nt, synthetic construct
  source 1..20: mol_type = other RNA
agaacctgaggagggggtgg

SEQ ID NO: 21029 - RNA, 20 nt, synthetic construct
  source 1..20: mol_type = other RNA
gagaacctgaggagggggtg

SEQ ID NO: 21030 - RNA, 20 nt, synthetic construct
  source 1..20: mol_type = other RNA
cccctcctcaggttctccca

SEQ ID NO: 21031 - RNA, 20 nt, synthetic construct
  source 1..20: mol_type = other RNA
gggagaacctgaggaggggg

SEQ ID NO: 21032 - RNA, 20 nt, synthetic construct
  source 1..20: mol_type = other RNA
cgtgggagaacctgaggagg

SEQ ID NO: 21033 - RNA, 20 nt, synthetic construct
  source 1..20: mol_type = other RNA
ccgtgggagaacctgaggag

SEQ ID NO: 21034 - RNA, 20 nt, synthetic construct
  source 1..20: mol_type = other RNA
gccgtgggagaacctgagga

SEQ ID NO: 21035 - RNA, 20 nt, synthetic construct
  source 1..20: mol_type = other RNA
tgccgtgggagaacctgagg

SEQ ID NO: 21036 - RNA, 20 nt, synthetic construct
  source 1..20: mol_type = other RNA
gtctgccgtgggagaacctg

SEQ ID NO: 21037 - RNA, 20 nt, synthetic construct
  source 1..20: mol_type = other RNA
gttctcccacggcagacctg

SEQ ID NO: 21038 - RNA, 20 nt, synthetic construct
  source 1..20: mol_type = other RNA
agaggccgcaggtctgccgt

SEQ ID NO: 21039 - RNA, 20 nt, synthetic construct
  source 1..20: mol_type = other RNA
aagaggccgcaggtctgccg

SEQ ID NO: 21040 - RNA, 20 nt, synthetic construct
  source 1..20: mol_type = other RNA
ggtgtgtgtgaagaggccgc

SEQ ID NO: 21041 - RNA, 20 nt, synthetic construct
  source 1..20: mol_type = other RNA
agaagatggtgtgtgtgaag

SEQ ID NO: 21042 - RNA, 20 nt, synthetic construct
  source 1..20: mol_type = other RNA
atcttctacaacgagtaccc

SEQ ID NO: 21043 - RNA, 20 nt, synthetic construct
  source 1..20: mol_type = other RNA
agggtactcgttgtagaaga

SEQ ID NO: 21044 - RNA, 20 nt, synthetic construct
  source 1..20: mol_type = other RNA
ccctggcggctccagtgagc

SEQ ID NO: 21045 - RNA, 20 nt, synthetic construct
  source 1..20: mol_type = other RNA
ccagctcactggagccgcca

SEQ ID NO: 21046 - RNA, 20 nt, synthetic construct
  source 1..20: mol_type = other RNA
tccagctcactggagccgcc

SEQ ID NO: 21047 - RNA, 20 nt, synthetic construct
  source 1..20: mol_type = other RNA
gatgatcttgtccagctcac

SEQ ID NO: 21048 - RNA, 20 nt, synthetic construct
  source 1..20: mol_type = other RNA
agctggacaagatcatcaac

SEQ ID NO: 21049 - RNA, 20 nt, synthetic construct
  source 1..20: mol_type = other RNA
gctggacaagatcatcaacg

SEQ ID NO: 21050 - RNA, 20 nt, synthetic construct
  source 1..20: mol_type = other RNA
ctggacaagatcatcaacgg

SEQ ID NO: 21051 - RNA, 20 nt, synthetic construct
  source 1..20: mol_type = other RNA
caggattgaggagcacggtg

SEQ ID NO: 21052 - RNA, 20 nt, synthetic construct
  source 1..20: mol_type = other RNA
actcacaggattgaggagca

SEQ ID NO: 21053 - RNA, 20 nt, synthetic construct
  source 1..20: mol_type = other RNA
gtggagcactcacaggattg

SEQ ID NO: 21054 - RNA, 20 nt, synthetic construct
  source 1..20: mol_type = other RNA
tgtgagtgctccacagccca

SEQ ID NO: 21055 - RNA, 20 nt, synthetic construct
  source 1..20: mol_type = other RNA
atgggctgtggagcactcac

SEQ ID NO: 21056 - RNA, 20 nt, synthetic construct
  source 1..20: mol_type = other RNA
gctccacagcccatggctgc

SEQ ID NO: 21057 - RNA, 20 nt, synthetic construct
  source 1..20: mol_type = other RNA
gcccatggctgctggtgaga

SEQ ID NO: 21058 - RNA, 20 nt, synthetic construct
  source 1..20: mol_type = other RNA
cccatggctgctggtgagaa

SEQ ID NO: 21059 - RNA, 20 nt, synthetic construct
  source 1..20: mol_type = other RNA
ccatggctgctggtgagaag

SEQ ID NO: 21060 - RNA, 20 nt, synthetic construct
  source 1..20: mol_type = other RNA
cccttctcaccagcagccat

SEQ ID NO: 21061 - RNA, 20 nt, synthetic construct
  source 1..20: mol_type = other RNA
ccccttctcaccagcagcca

SEQ ID NO: 21062 - RNA, 20 nt, synthetic construct
  source 1..20: mol_type = other RNA
agcctgtctgcagctgacac

SEQ ID NO: 21063 - RNA, 20 nt, synthetic construct
  source 1..20: mol_type = other RNA
agcctgtgtcagctgcagac

SEQ ID NO: 21064 - RNA, 20 nt, synthetic construct
  source 1..20: mol_type = other RNA
tgcagctgacacaggcttcc

SEQ ID NO: 21065 - RNA, 20 nt, synthetic construct
  source 1..20: mol_type = other RNA
gacacaggcttcctggagcc

SEQ ID NO: 21066 - RNA, 20 nt, synthetic construct
  source 1..20: mol_type = other RNA
aggcttcctggagccaggaa

SEQ ID NO: 21067 - RNA, 20 nt, synthetic construct
  source 1..20: mol_type = other RNA
ggcttcctggagccaggaaa

SEQ ID NO: 21068 - RNA, 20 nt, synthetic construct
  source 1..20: mol_type = other RNA
ttcctggagccaggaaaggg

SEQ ID NO: 21069 - RNA, 20 nt, synthetic construct
  source 1..20: mol_type = other RNA
ggagccaggaaagggtggag

SEQ ID NO: 21070 - RNA, 20 nt, synthetic construct
  source 1..20: mol_type = other RNA
ctccaccctttcctggctcc

SEQ ID NO: 21071 - RNA, 20 nt, synthetic construct
  source 1..20: mol_type = other RNA
catgcctctccaccctttcc

SEQ ID NO: 21072 - RNA, 20 nt, synthetic construct
  source 1..20: mol_type = other RNA
gagaggcatgagtgagtgcc

SEQ ID NO: 21073 - RNA, 20 nt, synthetic construct
  source 1..20: mol_type = other RNA
atgagtgagtgcctggcagt

SEQ ID NO: 21074 - RNA, 20 nt, synthetic construct
  source 1..20: mol_type = other RNA
tgagtgagtgcctggcagtt

SEQ ID NO: 21075 - RNA, 20 nt, synthetic construct
  source 1..20: mol_type = other RNA
gcaaggctcctgatgaccag

SEQ ID NO: 21076 - RNA, 20 nt, synthetic construct
  source 1..20: mol_type = other RNA
atcaggagccttgcaagcta

SEQ ID NO: 21077 - RNA, 20 nt, synthetic construct
  source 1..20: mol_type = other RNA
ggagccttgcaagctaaggc

SEQ ID NO: 21078 - RNA, 20 nt, synthetic construct
  source 1..20: mol_type = other RNA
gagccttgcaagctaaggca

SEQ ID NO: 21079 - RNA, 20 nt, synthetic construct
  source 1..20: mol_type = other RNA
tgaccctgccttagcttgca

SEQ ID NO: 21080 - RNA, 20 nt, synthetic construct
  source 1..20: mol_type = other RNA
aagctaaggcagggtcagaa

SEQ ID NO: 21081 - RNA, 20 nt, synthetic construct
  source 1..20: mol_type = other RNA
agggtcagaagggtcagagt

SEQ ID NO: 21082 - RNA, 20 nt, synthetic construct
  source 1..20: mol_type = other RNA
gtcagaagggtcagagttgg

SEQ ID NO: 21083 - RNA, 20 nt, synthetic construct
  source 1..20: mol_type = other RNA
aagggtcagagttggcggtg

SEQ ID NO: 21084 - RNA, 20 nt, synthetic construct
  source 1..20: mol_type = other RNA
agggtcagagttggcggtga

SEQ ID NO: 21085 - RNA, 20 nt, synthetic construct
  source 1..20: mol_type = other RNA
gtcagagttggcggtgaggg

SEQ ID NO: 21086 - RNA, 20 nt, synthetic construct
  source 1..20: mol_type = other RNA
gagggtggctcagacactga

SEQ ID NO: 21087 - RNA, 20 nt, synthetic construct
  source 1..20: mol_type = other RNA
agggtggctcagacactgat

SEQ ID NO: 21088 - RNA, 20 nt, synthetic construct
  source 1..20: mol_type = other RNA
gcctctctcctcccctcccc

SEQ ID NO: 21089 - RNA, 20 nt, synthetic construct
  source 1..20: mol_type = other RNA
gggaggggaggagagaggca

SEQ ID NO: 21090 - RNA, 20 nt, synthetic construct
  source 1..20: mol_type = other RNA
ggggaggggaggagagaggc

SEQ ID NO: 21091 - RNA, 20 nt, synthetic construct
  source 1..20: mol_type = other RNA
tccaggggaggggaggagag

SEQ ID NO: 21092 - RNA, 20 nt, synthetic construct
  source 1..20: mol_type = other RNA
gatctgctccaggggagggg

SEQ ID NO: 21093 - RNA, 20 nt, synthetic construct
  source 1..20: mol_type = other RNA
gctgatctgctccaggggag

SEQ ID NO: 21094 - RNA, 20 nt, synthetic construct
  source 1..20: mol_type = other RNA
tgctgatctgctccagggga

SEQ ID NO: 21095 - RNA, 20 nt, synthetic construct
  source 1..20: mol_type = other RNA
atgctgatctgctccagggg

SEQ ID NO: 21096 - RNA, 20 nt, synthetic construct
  source 1..20: mol_type = other RNA
aagatgctgatctgctccag

SEQ ID NO: 21097 - RNA, 20 nt, synthetic construct
  source 1..20: mol_type = other RNA
gaagatgctgatctgctcca

SEQ ID NO: 21098 - RNA, 20 nt, synthetic construct
  source 1..20: mol_type = other RNA
tgaagatgctgatctgctcc

SEQ ID NO: 21099 - RNA, 20 nt, synthetic construct
  source 1..20: mol_type = other RNA
atgacgcacctgtccaacta

SEQ ID NO: 21100 - RNA, 20 nt, synthetic construct
  source 1..20: mol_type = other RNA
tgacgcacctgtccaactat

SEQ ID NO: 21101 - RNA, 20 nt, synthetic construct
  source 1..20: mol_type = other RNA
ggtcattcccatagttggac

SEQ ID NO: 21102 - RNA, 20 nt, synthetic construct
  source 1..20: mol_type = other RNA
caactatgggaatgaccgcc

SEQ ID NO: 21103 - RNA, 20 nt, synthetic construct
  source 1..20: mol_type = other RNA
aactatgggaatgaccgcct

SEQ ID NO: 21104 - RNA, 20 nt, synthetic construct
  source 1..20: mol_type = other RNA
caggcggtcattcccatagt

SEQ ID NO: 21105 - RNA, 20 nt, synthetic construct
  source 1..20: mol_type = other RNA
tgaaggtgtacaggcccagg

SEQ ID NO: 21106 - RNA, 20 nt, synthetic construct
  source 1..20: mol_type = other RNA
gcttgaaggtgtacaggccc

SEQ ID NO: 21107 - RNA, 20 nt, synthetic construct
  source 1..20: mol_type = other RNA
cctgtacaccttcaagcacc

SEQ ID NO: 21108 - RNA, 20 nt, synthetic construct
  source 1..20: mol_type = other RNA
ccaggtgcttgaaggtgtac

SEQ ID NO: 21109 - RNA, 20 nt, synthetic construct
  source 1..20: mol_type = other RNA
gaagcgcaccaggtgcttga

SEQ ID NO: 21110 - RNA, 20 nt, synthetic construct
  source 1..20: mol_type = other RNA
tggtgcgcttcctgcactcc

SEQ ID NO: 21111 - RNA, 20 nt, synthetic construct
  source 1..20: mol_type = other RNA
aggagtgcaggaagcgcacc

SEQ ID NO: 21112 - RNA, 20 nt, synthetic construct
  source 1..20: mol_type = other RNA
tgcactcctggacgaacctc

SEQ ID NO: 21113 - RNA, 20 nt, synthetic construct
  source 1..20: mol_type = other RNA
ggaggttcgtccaggagtgc

SEQ ID NO: 21114 - RNA, 20 nt, synthetic construct
  source 1..20: mol_type = other RNA
ctgcagccggaggttcgtcc

SEQ ID NO: 21115 - RNA, 20 nt, synthetic construct
  source 1..20: mol_type = other RNA
ggggcagtgtctgcagccgg

SEQ ID NO: 21116 - RNA, 20 nt, synthetic construct
  source 1..20: mol_type = other RNA
cagggggcagtgtctgcagc

SEQ ID NO: 21117 - RNA, 20 nt, synthetic construct
  source 1..20: mol_type = other RNA
gacactgccccctgtgcagt

SEQ ID NO: 21118 - RNA, 20 nt, synthetic construct
  source 1..20: mol_type = other RNA
ttctgcgccaactgcacagg

SEQ ID NO: 21119 - RNA, 20 nt, synthetic construct
  source 1..20: mol_type = other RNA
cttctgcgccaactgcacag

SEQ ID NO: 21120 - RNA, 20 nt, synthetic construct
  source 1..20: mol_type = other RNA
acttctgcgccaactgcaca

SEQ ID NO: 21121 - RNA, 20 nt, synthetic construct
  source 1..20: mol_type = other RNA
tacttctgcgccaactgcac

SEQ ID NO: 21122 - RNA, 20 nt, synthetic construct
  source 1..20: mol_type = other RNA
gtacttccagatcttctccg

SEQ ID NO: 21123 - RNA, 20 nt, synthetic construct
  source 1..20: mol_type = other RNA
ccagatcttctccgaggaga

SEQ ID NO: 21124 - RNA, 20 nt, synthetic construct
  source 1..20: mol_type = other RNA
ccttctcctcggagaagatc

SEQ ID NO: 21125 - RNA, 20 nt, synthetic construct
  source 1..20: mol_type = other RNA
ccgaggagaaggacccgctc

SEQ ID NO: 21126 - RNA, 20 nt, synthetic construct
  source 1..20: mol_type = other RNA
ggagaaggacccgctctggc

SEQ ID NO: 21127 - RNA, 20 nt, synthetic construct
  source 1..20: mol_type = other RNA
ccagagcgggtccttctcct

SEQ ID NO: 21128 - RNA, 20 nt, synthetic construct
  source 1..20: mol_type = other RNA
gaaggacccgctctggcagg

SEQ ID NO: 21129 - RNA, 20 nt, synthetic construct
  source 1..20: mol_type = other RNA
aaggacccgctctggcaggt

SEQ ID NO: 21130 - RNA, 20 nt, synthetic construct
  source 1..20: mol_type = other RNA
aggacccgctctggcaggtg

SEQ ID NO: 21131 - RNA, 20 nt, synthetic construct
  source 1..20: mol_type = other RNA
ggacccgctctggcaggtgg

SEQ ID NO: 21132 - RNA, 20 nt, synthetic construct
  source 1..20: mol_type = other RNA
gacccgctctggcaggtggg

SEQ ID NO: 21133 - RNA, 20 nt, synthetic construct
  source 1..20: mol_type = other RNA
cgctctggcaggtggggggc

SEQ ID NO: 21134 - RNA, 20 nt, synthetic construct
  source 1..20: mol_type = other RNA
gctctggcaggtggggggct

SEQ ID NO: 21135 - RNA, 20 nt, synthetic construct
  source 1..20: mol_type = other RNA
agccccccacctgccagagc

SEQ ID NO: 21136 - RNA, 20 nt, synthetic construct
  source 1..20: mol_type = other RNA
cagccccccacctgccagag

SEQ ID NO: 21137 - RNA, 20 nt, synthetic construct
  source 1..20: mol_type = other RNA
aggtggggggctgggcagcc

SEQ ID NO: 21138 - RNA, 20 nt, synthetic construct
  source 1..20: mol_type = other RNA
ggtggggggctgggcagcct

SEQ ID NO: 21139 - RNA, 20 nt, synthetic construct
  source 1..20: mol_type = other RNA
gggggctgggcagcctgggc

SEQ ID NO: 21140 - RNA, 20 nt, synthetic construct
  source 1..20: mol_type = other RNA
cagcctgggcaggttgctac

SEQ ID NO: 21141 - RNA, 20 nt, synthetic construct
  source 1..20: mol_type = other RNA
agcctgggcaggttgctaca

SEQ ID NO: 21142 - RNA, 20 nt, synthetic construct
  source 1..20: mol_type = other RNA
tgggcaggttgctacaggga

SEQ ID NO: 21143 - RNA, 20 nt, synthetic construct
  source 1..20: mol_type = other RNA
atccctgtagcaacctgccc

SEQ ID NO: 21144 - RNA, 20 nt, synthetic construct
  source 1..20: mol_type = other RNA
gatggaacgccaccactcac

SEQ ID NO: 21145 - RNA, 20 nt, synthetic construct
  source 1..20: mol_type = other RNA
gagtgtgtgcctgtgagtgg

SEQ ID NO: 21146 - RNA, 20 nt, synthetic construct
  source 1..20: mol_type = other RNA
ctggagtgtgtgcctgtgag

SEQ ID NO: 21147 - RNA, 20 nt, synthetic construct
  source 1..20: mol_type = other RNA
acaggcacacactccagata

SEQ ID NO: 21148 - RNA, 20 nt, synthetic construct
  source 1..20: mol_type = other RNA
acactccagatatggactca

SEQ ID NO: 21149 - RNA, 20 nt, synthetic construct
  source 1..20: mol_type = other RNA
ctgagccttgagtccatatc

SEQ ID NO: 21150 - RNA, 20 nt, synthetic construct
  source 1..20: mol_type = other RNA
gcgagagtgtgaaggcatga

SEQ ID NO: 21151 - RNA, 20 nt, synthetic construct
  source 1..20: mol_type = other RNA
acattcgagcgagagtgtga

SEQ ID NO: 21152 - RNA, 20 nt, synthetic construct
  source 1..20: mol_type = other RNA
catgtaggtatcatgcccat

SEQ ID NO: 21153 - RNA, 20 nt, synthetic construct
  source 1..20: mol_type = other RNA
atgtaggtatcatgcccatt

SEQ ID NO: 21154 - RNA, 20 nt, synthetic construct
  source 1..20: mol_type = other RNA
atcatgcccattgggctgta

SEQ ID NO: 21155 - RNA, 20 nt, synthetic construct
  source 1..20: mol_type = other RNA
tcatgcccattgggctgtaa

SEQ ID NO: 21156 - RNA, 20 nt, synthetic construct
  source 1..20: mol_type = other RNA
tgtggcccttacagcccaat

SEQ ID NO: 21157 - RNA, 20 nt, synthetic construct
  source 1..20: mol_type = other RNA
atgtggcccttacagcccaa

SEQ ID NO: 21158 - RNA, 20 nt, synthetic construct
  source 1..20: mol_type = other RNA
ggccacatatccatgtgcag

SEQ ID NO: 21159 - RNA, 20 nt, synthetic construct
  source 1..20: mol_type = other RNA
gccacatatccatgtgcagt

SEQ ID NO: 21160 - RNA, 20 nt, synthetic construct
  source 1..20: mol_type = other RNA
tcccactgcacatggatatg

SEQ ID NO: 21161 - RNA, 20 nt, synthetic construct
  source 1..20: mol_type = other RNA
tgcagtgggagtccactgac

SEQ ID NO: 21162 - RNA, 20 nt, synthetic construct
  source 1..20: mol_type = other RNA
gcagtgggagtccactgact

SEQ ID NO: 21163 - RNA, 20 nt, synthetic construct
  source 1..20: mol_type = other RNA
ggagtccactgactgggttc

SEQ ID NO: 21164 - RNA, 20 nt, synthetic construct
  source 1..20: mol_type = other RNA
gagtccactgactgggttct

SEQ ID NO: 21165 - RNA, 20 nt, synthetic construct
  source 1..20: mol_type = other RNA
agtccactgactgggttctg

SEQ ID NO: 21166 - RNA, 20 nt, synthetic construct
  source 1..20: mol_type = other RNA
gcgccccagaacccagtcag

SEQ ID NO: 21167 - RNA, 20 nt, synthetic construct
  source 1..20: mol_type = other RNA
aacagtggaagggatgtgtg

SEQ ID NO: 21168 - RNA, 20 nt, synthetic construct
  source 1..20: mol_type = other RNA
caacagtggaagggatgtgt

SEQ ID NO: 21169 - RNA, 20 nt, synthetic construct
  source 1..20: mol_type = other RNA
acaacagtggaagggatgtg

SEQ ID NO: 21170 - RNA, 20 nt, synthetic construct
  source 1..20: mol_type = other RNA
atcccttccactgttgtttt

SEQ ID NO: 21171 - RNA, 20 nt, synthetic construct
  source 1..20: mol_type = other RNA
gtcctaaaacaacagtggaa

SEQ ID NO: 21172 - RNA, 20 nt, synthetic construct
  source 1..20: mol_type = other RNA
ggtcctaaaacaacagtgga

SEQ ID NO: 21173 - RNA, 20 nt, synthetic construct
  source 1..20: mol_type = other RNA
gttgttttaggacccctgcg

SEQ ID NO: 21174 - RNA, 20 nt, synthetic construct
  source 1..20: mol_type = other RNA
tgtgacgtttgtcctcgcag

SEQ ID NO: 21175 - RNA, 20 nt, synthetic construct
  source 1..20: mol_type = other RNA
ttgtgacgtttgtcctcgca

SEQ ID NO: 21176 - RNA, 20 nt, synthetic construct
  source 1..20: mol_type = other RNA
tttgtgacgtttgtcctcgc

SEQ ID NO: 21177 - RNA, 20 nt, synthetic construct
  source 1..20: mol_type = other RNA
acaaacgtcacaaagacatc

SEQ ID NO: 21178 - RNA, 20 nt, synthetic construct
  source 1..20: mol_type = other RNA
tcacaaagacatctggtcca

SEQ ID NO: 21179 - RNA, 20 nt, synthetic construct
  source 1..20: mol_type = other RNA
gcggtcacacgtcttctcct

SEQ ID NO: 21180 - RNA, 20 nt, synthetic construct
  source 1..20: mol_type = other RNA
ttcccaaagctcctcatcat

SEQ ID NO: 21181 - RNA, 20 nt, synthetic construct
  source 1..20: mol_type = other RNA
tgatgaggagctttgggaag

SEQ ID NO: 21182 - RNA, 20 nt, synthetic construct
  source 1..20: mol_type = other RNA
ggccgatgatgaggagcttt

SEQ ID NO: 21183 - RNA, 20 nt, synthetic construct
  source 1..20: mol_type = other RNA
gggccgatgatgaggagctt

SEQ ID NO: 21184 - RNA, 20 nt, synthetic construct
  source 1..20: mol_type = other RNA
atcatcggcccccagaaaac

SEQ ID NO: 21185 - RNA, 20 nt, synthetic construct
  source 1..20: mol_type = other RNA
ttttctgggggccgatgatg

SEQ ID NO: 21186 - RNA, 20 nt, synthetic construct
  source 1..20: mol_type = other RNA
tcggcccccagaaaacaggc

SEQ ID NO: 21187 - RNA, 20 nt, synthetic construct
  source 1..20: mol_type = other RNA
gagacctgcctgttttctgg

SEQ ID NO: 21188 - RNA, 20 nt, synthetic construct
  source 1..20: mol_type = other RNA
agagacctgcctgttttctg

SEQ ID NO: 21189 - RNA, 20 nt, synthetic construct
  source 1..20: mol_type = other RNA
gagagacctgcctgttttct

SEQ ID NO: 21190 - RNA, 20 nt, synthetic construct
  source 1..20: mol_type = other RNA
agagagacctgcctgttttc

SEQ ID NO: 21191 - RNA, 20 nt, synthetic construct
  source 1..20: mol_type = other RNA
agcaggcagttggggaagct

SEQ ID NO: 21192 - RNA, 20 nt, synthetic construct
  source 1..20: mol_type = other RNA
gctgagacagcaggcagttg

SEQ ID NO: 21193 - RNA, 20 nt, synthetic construct
  source 1..20: mol_type = other RNA
ggctgagacagcaggcagtt

SEQ ID NO: 21194 - RNA, 20 nt, synthetic construct
  source 1..20: mol_type = other RNA
tggctgagacagcaggcagt

SEQ ID NO: 21195 - RNA, 20 nt, synthetic construct
  source 1..20: mol_type = other RNA
aattctgtggctgagacagc

SEQ ID NO: 21196 - RNA, 20 nt, synthetic construct
  source 1..20: mol_type = other RNA
gtctcagccacagaattctg

SEQ ID NO: 21197 - RNA, 20 nt, synthetic construct
  source 1..20: mol_type = other RNA
aggcagtcctcagaattctg

SEQ ID NO: 21198 - RNA, 20 nt, synthetic construct
  source 1..20: mol_type = other RNA
ttctgaggactgccttgccc

SEQ ID NO: 21199 - RNA, 20 nt, synthetic construct
  source 1..20: mol_type = other RNA
ccttgccctggccccactcc

SEQ ID NO: 21200 - RNA, 20 nt, synthetic construct
  source 1..20: mol_type = other RNA
ccgggagtggggccagggca

SEQ ID NO: 21201 - RNA, 20 nt, synthetic construct
  source 1..20: mol_type = other RNA
attatccgggagtggggcca

SEQ ID NO: 21202 - RNA, 20 nt, synthetic construct
  source 1..20: mol_type = other RNA
aattatccgggagtggggcc

SEQ ID NO: 21203 - RNA, 20 nt, synthetic construct
  source 1..20: mol_type = other RNA
gagcaaattatccgggagtg

SEQ ID NO: 21204 - RNA, 20 nt, synthetic construct
  source 1..20: mol_type = other RNA
ggagcaaattatccgggagt

SEQ ID NO: 21205 - RNA, 20 nt, synthetic construct
  source 1..20: mol_type = other RNA
gggagcaaattatccgggag

SEQ ID NO: 21206 - RNA, 20 nt, synthetic construct
  source 1..20: mol_type = other RNA
aaagagggagcaaattatcc

SEQ ID NO: 21207 - RNA, 20 nt, synthetic construct
  source 1..20: mol_type = other RNA
gaaagagggagcaaattatc

SEQ ID NO: 21208 - RNA, 20 nt, synthetic construct
  source 1..20: mol_type = other RNA
ctccctctttcccaggaagt

SEQ ID NO: 21209 - RNA, 20 nt, synthetic construct
  source 1..20: mol_type = other RNA
agaaaggcagagaccttccc

SEQ ID NO: 21210 - RNA, 20 nt, synthetic construct
  source 1..20: mol_type = other RNA
ggaaggtctctgcctttctc

SEQ ID NO: 21211 - RNA, 20 nt, synthetic construct
  source 1..20: mol_type = other RNA
accttcccaggagcccccag

SEQ ID NO: 21212 - RNA, 20 nt, synthetic construct
  source 1..20: mol_type = other RNA
ccttcccaggagcccccagt

SEQ ID NO: 21213 - RNA, 20 nt, synthetic construct
  source 1..20: mol_type = other RNA
cccactgggggctcctggga

SEQ ID NO: 21214 - RNA, 20 nt, synthetic construct
  source 1..20: mol_type = other RNA
caggagcccccagtgggtcg

SEQ ID NO: 21215 - RNA, 20 nt, synthetic construct
  source 1..20: mol_type = other RNA
aggagcccccagtgggtcgt

SEQ ID NO: 21216 - RNA, 20 nt, synthetic construct
  source 1..20: mol_type = other RNA
ggagcccccagtgggtcgtg

SEQ ID NO: 21217 - RNA, 20 nt, synthetic construct
  source 1..20: mol_type = other RNA
acgacccactgggggctcct

SEQ ID NO: 21218 - RNA, 20 nt, synthetic construct
  source 1..20: mol_type = other RNA
cacgacccactgggggctcc

SEQ ID NO: 21219 - RNA, 20 nt, synthetic construct
  source 1..20: mol_type = other RNA
ccagtgggtcgtggggagct

SEQ ID NO: 21220 - RNA, 20 nt, synthetic construct
  source 1..20: mol_type = other RNA
agctccccacgacccactgg

SEQ ID NO: 21221 - RNA, 20 nt, synthetic construct
  source 1..20: mol_type = other RNA
tagctccccacgacccactg

SEQ ID NO: 21222 - RNA, 20 nt, synthetic construct
  source 1..20: mol_type = other RNA
ctagctccccacgacccact

SEQ ID NO: 21223 - RNA, 20 nt, synthetic construct
  source 1..20: mol_type = other RNA
cctagctccccacgacccac

SEQ ID NO: 21224 - RNA, 20 nt, synthetic construct
  source 1..20: mol_type = other RNA
agaacccagactctatcttt

SEQ ID NO: 21225 - RNA, 20 nt, synthetic construct
  source 1..20: mol_type = other RNA
aaagatagagtctgggttct

SEQ ID NO: 21226 - RNA, 20 nt, synthetic construct
  source 1..20: mol_type = other RNA
aaaagatagagtctgggttc

SEQ ID NO: 21227 - RNA, 20 nt, synthetic construct
  source 1..20: mol_type = other RNA
cccagactctatcttttggc

SEQ ID NO: 21228 - RNA, 20 nt, synthetic construct
  source 1..20: mol_type = other RNA
ccagactctatcttttggct

SEQ ID NO: 21229 - RNA, 20 nt, synthetic construct
  source 1..20: mol_type = other RNA
cagactctatcttttggctg

SEQ ID NO: 21230 - RNA, 20 nt, synthetic construct
  source 1..20: mol_type = other RNA
agactctatcttttggctgg

SEQ ID NO: 21231 - RNA, 20 nt, synthetic construct
  source 1..20: mol_type = other RNA
ccagccaaaagatagagtct

SEQ ID NO: 21232 - RNA, 20 nt, synthetic construct
  source 1..20: mol_type = other RNA
cccagccaaaagatagagtc

SEQ ID NO: 21233 - RNA, 20 nt, synthetic construct
  source 1..20: mol_type = other RNA
tctatcttttggctgggggc

SEQ ID NO: 21234 - RNA, 20 nt, synthetic construct
  source 1..20: mol_type = other RNA
ctatcttttggctgggggct

SEQ ID NO: 21235 - RNA, 20 nt, synthetic construct
  source 1..20: mol_type = other RNA
tttggctgggggctgggccc

SEQ ID NO: 21236 - RNA, 20 nt, synthetic construct
  source 1..20: mol_type = other RNA
ttggctgggggctgggccct

SEQ ID NO: 21237 - RNA, 20 nt, synthetic construct
  source 1..20: mol_type = other RNA
ggggctgggccctgggtctc

SEQ ID NO: 21238 - RNA, 20 nt, synthetic construct
  source 1..20: mol_type = other RNA
gggtagacacctgagaccca

SEQ ID NO: 21239 - RNA, 20 nt, synthetic construct
  source 1..20: mol_type = other RNA
agggtagacacctgagaccc

SEQ ID NO: 21240 - RNA, 20 nt, synthetic construct
  source 1..20: mol_type = other RNA
caggtgtctaccctccccac

SEQ ID NO: 21241 - RNA, 20 nt, synthetic construct
  source 1..20: mol_type = other RNA
ggcagtggtgcctgtgggga

SEQ ID NO: 21242 - RNA, 20 nt, synthetic construct
  source 1..20: mol_type = other RNA
gggcagtggtgcctgtgggg

SEQ ID NO: 21243 - RNA, 20 nt, synthetic construct
  source 1..20: mol_type = other RNA
agagggcagtggtgcctgtg

SEQ ID NO: 21244 - RNA, 20 nt, synthetic construct
  source 1..20: mol_type = other RNA
tagagggcagtggtgcctgt

SEQ ID NO: 21245 - RNA, 20 nt, synthetic construct
  source 1..20: mol_type = other RNA
gtagagggcagtggtgcctg

SEQ ID NO: 21246 - RNA, 20 nt, synthetic construct
  source 1..20: mol_type = other RNA
cactgccctctacctgttcc

SEQ ID NO: 21247 - RNA, 20 nt, synthetic construct
  source 1..20: mol_type = other RNA
actgccctctacctgttcct

SEQ ID NO: 21248 - RNA, 20 nt, synthetic construct
  source 1..20: mol_type = other RNA
caggaacaggtagagggcag

SEQ ID NO: 21249 - RNA, 20 nt, synthetic construct
  source 1..20: mol_type = other RNA
catgcccaggaacaggtaga

SEQ ID NO: 21250 - RNA, 20 nt, synthetic construct
  source 1..20: mol_type = other RNA
gcatgcccaggaacaggtag

SEQ ID NO: 21251 - RNA, 20 nt, synthetic construct
  source 1..20: mol_type = other RNA
cagggtgcatgcccaggaac

SEQ ID NO: 21252 - RNA, 20 nt, synthetic construct
  source 1..20: mol_type = other RNA
ttaggtcagggtgcatgccc

SEQ ID NO: 21253 - RNA, 20 nt, synthetic construct
  source 1..20: mol_type = other RNA
ggtagttgctgcttaggtca

SEQ ID NO: 21254 - RNA, 20 nt, synthetic construct
  source 1..20: mol_type = other RNA
gggtagttgctgcttaggtc

SEQ ID NO: 21255 - RNA, 20 nt, synthetic construct
  source 1..20: mol_type = other RNA
agctggggtagttgctgctt

SEQ ID NO: 21256 - RNA, 20 nt, synthetic construct
  source 1..20: mol_type = other RNA
ccccagctctgagacctttg

SEQ ID NO: 21257 - RNA, 20 nt, synthetic construct
  source 1..20: mol_type = other RNA
cctcaaaggtctcagagctg

SEQ ID NO: 21258 - RNA, 20 nt, synthetic construct
  source 1..20: mol_type = other RNA
tcctcaaaggtctcagagct

SEQ ID NO: 21259 - RNA, 20 nt, synthetic construct
  source 1..20: mol_type = other RNA
ctcctcaaaggtctcagagc

SEQ ID NO: 21260 - RNA, 20 nt, synthetic construct
  source 1..20: mol_type = other RNA
gaggagatccagttttttaa

SEQ ID NO: 21261 - RNA, 20 nt, synthetic construct
  source 1..20: mol_type = other RNA
agttgtggccattaaaaaac

SEQ ID NO: 21262 - RNA, 20 nt, synthetic construct
  source 1..20: mol_type = other RNA
aatggccacaactatcacaa

SEQ ID NO: 21263 - RNA, 20 nt, synthetic construct
  source 1..20: mol_type = other RNA
cgatgcctttgtgatagttg

SEQ ID NO: 21264 - RNA, 20 nt, synthetic construct
  source 1..20: mol_type = other RNA
aaaggcatcgactggtgagt

SEQ ID NO: 21265 - RNA, 20 nt, synthetic construct
  source 1..20: mol_type = other RNA
gttggcctttctgtccacag

SEQ ID NO: 21266 - RNA, 20 nt, synthetic construct
  source 1..20: mol_type = other RNA
ttggcctttctgtccacagc

SEQ ID NO: 21267 - RNA, 20 nt, synthetic construct
  source 1..20: mol_type = other RNA
cctttctgtccacagcggga

SEQ ID NO: 21268 - RNA, 20 nt, synthetic construct
  source 1..20: mol_type = other RNA
ctttctgtccacagcgggac

SEQ ID NO: 21269 - RNA, 20 nt, synthetic construct
  source 1..20: mol_type = other RNA
ccgtcccgctgtggacagaa

SEQ ID NO: 21270 - RNA, 20 nt, synthetic construct
  source 1..20: mol_type = other RNA
atggccttcccgtcccgctg

SEQ ID NO: 21271 - RNA, 20 nt, synthetic construct
  source 1..20: mol_type = other RNA
cgggacgggaaggccatcct

SEQ ID NO: 21272 - RNA, 20 nt, synthetic construct
  source 1..20: mol_type = other RNA
gggacgggaaggccatcctg

SEQ ID NO: 21273 - RNA, 20 nt, synthetic construct
  source 1..20: mol_type = other RNA
aggccatcctggggcctccc

SEQ ID NO: 21274 - RNA, 20 nt, synthetic construct
  source 1..20: mol_type = other RNA
actcctgggaggccccagga

SEQ ID NO: 21275 - RNA, 20 nt, synthetic construct
  source 1..20: mol_type = other RNA
ggcctcccaggagtctgctg

SEQ ID NO: 21276 - RNA, 20 nt, synthetic construct
  source 1..20: mol_type = other RNA
ggccacagcagactcctggg

SEQ ID NO: 21277 - RNA, 20 nt, synthetic construct
  source 1..20: mol_type = other RNA
tgtggccacagcagactcct

SEQ ID NO: 21278 - RNA, 20 nt, synthetic construct
  source 1..20: mol_type = other RNA
ctgtggccacagcagactcc

SEQ ID NO: 21279 - RNA, 20 nt, synthetic construct
  source 1..20: mol_type = other RNA
tggccacagcaggaagcagc

SEQ ID NO: 21280 - RNA, 20 nt, synthetic construct
  source 1..20: mol_type = other RNA
gctccagctgcttcctgctg

SEQ ID NO: 21281 - RNA, 20 nt, synthetic construct
  source 1..20: mol_type = other RNA
cagctgtcattcctgtaaac

SEQ ID NO: 21282 - RNA, 20 nt, synthetic construct
  source 1..20: mol_type = other RNA
agctgtcattcctgtaaaca

SEQ ID NO: 21283 - RNA, 20 nt, synthetic construct
  source 1..20: mol_type = other RNA
agcttcccacttgctctctg

SEQ ID NO: 21284 - RNA, 20 nt, synthetic construct
  source 1..20: mol_type = other RNA
aatgtcctcagagagcaagt

SEQ ID NO: 21285 - RNA, 20 nt, synthetic construct
  source 1..20: mol_type = other RNA
gaatgtcctcagagagcaag

SEQ ID NO: 21286 - RNA, 20 nt, synthetic construct
  source 1..20: mol_type = other RNA
agcacaagggcgaggcactg

SEQ ID NO: 21287 - RNA, 20 nt, synthetic construct
  source 1..20: mol_type = other RNA
cagcacaagggcgaggcact

SEQ ID NO: 21288 - RNA, 20 nt, synthetic construct
  source 1..20: mol_type = other RNA
gcagcacaagggcgaggcac

SEQ ID NO: 21289 - RNA, 20 nt, synthetic construct
  source 1..20: mol_type = other RNA
gggaatgcagcacaagggcg

SEQ ID NO: 21290 - RNA, 20 nt, synthetic construct
  source 1..20: mol_type = other RNA
gctaagggaatgcagcacaa

SEQ ID NO: 21291 - RNA, 20 nt, synthetic construct
  source 1..20: mol_type = other RNA
ggctaagggaatgcagcaca

SEQ ID NO: 21292 - RNA, 20 nt, synthetic construct
  source 1..20: mol_type = other RNA
actcatgaggagggggctaa

SEQ ID NO: 21293 - RNA, 20 nt, synthetic construct
  source 1..20: mol_type = other RNA
aactcatgaggagggggcta

SEQ ID NO: 21294 - RNA, 20 nt, synthetic construct
  source 1..20: mol_type = other RNA
agacaaaactcatgaggagg

SEQ ID NO: 21295 - RNA, 20 nt, synthetic construct
  source 1..20: mol_type = other RNA
cagacaaaactcatgaggag

SEQ ID NO: 21296 - RNA, 20 nt, synthetic construct
  source 1..20: mol_type = other RNA
acagacaaaactcatgagga

SEQ ID NO: 21297 - RNA, 20 nt, synthetic construct
  source 1..20: mol_type = other RNA
cacagacaaaactcatgagg

SEQ ID NO: 21298 - RNA, 20 nt, synthetic construct
  source 1..20: mol_type = other RNA
gctcacagacaaaactcatg

SEQ ID NO: 21299 - RNA, 20 nt, synthetic construct
  source 1..20: mol_type = other RNA
ttgtctgtgagccgcctctc

SEQ ID NO: 21300 - RNA, 20 nt, synthetic construct
  source 1..20: mol_type = other RNA
tgtctgtgagccgcctctct

SEQ ID NO: 21301 - RNA, 20 nt, synthetic construct
  source 1..20: mol_type = other RNA
cgcctctctgggcttcctgc

SEQ ID NO: 21302 - RNA, 20 nt, synthetic construct
  source 1..20: mol_type = other RNA
ctgcaggaagcccagagagg

SEQ ID NO: 21303 - RNA, 20 nt, synthetic construct
  source 1..20: mol_type = other RNA
tacctgcaggaagcccagag

SEQ ID NO: 21304 - RNA, 20 nt, synthetic construct
  source 1..20: mol_type = other RNA
gaagaactccatgtacctgc

SEQ ID NO: 21305 - RNA, 20 nt, synthetic construct
  source 1..20: mol_type = other RNA
aggtggtgttggaagggatg

SEQ ID NO: 21306 - RNA, 20 nt, synthetic construct
  source 1..20: mol_type = other RNA
gaggtggtgttggaagggat

SEQ ID NO: 21307 - RNA, 20 nt, synthetic construct
  source 1..20: mol_type = other RNA
ggaggtggtgttggaaggga

SEQ ID NO: 21308 - RNA, 20 nt, synthetic construct
  source 1..20: mol_type = other RNA
agtcggaggtggtgttggaa

SEQ ID NO: 21309 - RNA, 20 nt, synthetic construct
  source 1..20: mol_type = other RNA
aagtcggaggtggtgttgga

SEQ ID NO: 21310 - RNA, 20 nt, synthetic construct
  source 1..20: mol_type = other RNA
gtagaagtcggaggtggtgt

SEQ ID NO: 21311 - RNA, 20 nt, synthetic construct
  source 1..20: mol_type = other RNA
ctcaaagtagaagtcggagg

SEQ ID NO: 21312 - RNA, 20 nt, synthetic construct
  source 1..20: mol_type = other RNA
tttctcaaagtagaagtcgg

SEQ ID NO: 21313 - RNA, 20 nt, synthetic construct
  source 1..20: mol_type = other RNA
gcttttctcaaagtagaagt

SEQ ID NO: 21314 - RNA, 20 nt, synthetic construct
  source 1..20: mol_type = other RNA
caactactttgattcagaag

SEQ ID NO: 21315 - RNA, 20 nt, synthetic construct
  source 1..20: mol_type = other RNA
cacttctgaatcaaagtagt

SEQ ID NO: 21316 - RNA, 20 nt, synthetic construct
  source 1..20: mol_type = other RNA
ttgattcagaagtggcgccc

SEQ ID NO: 21317 - RNA, 20 nt, synthetic construct
  source 1..20: mol_type = other RNA
attcagaagtggcgccccgg

SEQ ID NO: 21318 - RNA, 20 nt, synthetic construct
  source 1..20: mol_type = other RNA
ttcagaagtggcgccccggc

SEQ ID NO: 21319 - RNA, 20 nt, synthetic construct
  source 1..20: mol_type = other RNA
aagagggctgctgcccgccg

SEQ ID NO: 21320 - RNA, 20 nt, synthetic construct
  source 1..20: mol_type = other RNA
caagagggctgctgcccgcc

SEQ ID NO: 21321 - RNA, 20 nt, synthetic construct
  source 1..20: mol_type = other RNA
gcaagagggctgctgcccgc

SEQ ID NO: 21322 - RNA, 20 nt, synthetic construct
  source 1..20: mol_type = other RNA
agccctcttgcccaaagcca

SEQ ID NO: 21323 - RNA, 20 nt, synthetic construct
  source 1..20: mol_type = other RNA
gaccttggctttgggcaaga

SEQ ID NO: 21324 - RNA, 20 nt, synthetic construct
  source 1..20: mol_type = other RNA
ggaccttggctttgggcaag

SEQ ID NO: 21325 - RNA, 20 nt, synthetic construct
  source 1..20: mol_type = other RNA
atggtcaggaccttggcttt

SEQ ID NO: 21326 - RNA, 20 nt, synthetic construct
  source 1..20: mol_type = other RNA
gatggtcaggaccttggctt

SEQ ID NO: 21327 - RNA, 20 nt, synthetic construct
  source 1..20: mol_type = other RNA
gatgaggatggtcaggacct

SEQ ID NO: 21328 - RNA, 20 nt, synthetic construct
  source 1..20: mol_type = other RNA
gaccatcctcatcaaccccg

SEQ ID NO: 21329 - RNA, 20 nt, synthetic construct
  source 1..20: mol_type = other RNA
cggggttgatgaggatggtc

SEQ ID NO: 21330 - RNA, 20 nt, synthetic construct
  source 1..20: mol_type = other RNA
tcctcatcaaccccgcggac

SEQ ID NO: 21331 - RNA, 20 nt, synthetic construct
  source 1..20: mol_type = other RNA
cctcatcaaccccgcggacc

SEQ ID NO: 21332 - RNA, 20 nt, synthetic construct
  source 1..20: mol_type = other RNA
gtccgcggggttgatgagga

SEQ ID NO: 21333 - RNA, 20 nt, synthetic construct
  source 1..20: mol_type = other RNA
cccggtccgcggggttgatg

SEQ ID NO: 21334 - RNA, 20 nt, synthetic construct
  source 1..20: mol_type = other RNA
ccgcggaccgggcctattcc

SEQ ID NO: 21335 - RNA, 20 nt, synthetic construct
  source 1..20: mol_type = other RNA
aggaataggcccggtccgcg

SEQ ID NO: 21336 - RNA, 20 nt, synthetic construct
  source 1..20: mol_type = other RNA
caggaataggcccggtccgc

SEQ ID NO: 21337 - RNA, 20 nt, synthetic construct
  source 1..20: mol_type = other RNA
ccaggaataggcccggtccg

SEQ ID NO: 21338 - RNA, 20 nt, synthetic construct
  source 1..20: mol_type = other RNA
ccgggcctattcctggtacc

SEQ ID NO: 21339 - RNA, 20 nt, synthetic construct
  source 1..20: mol_type = other RNA
cctggtaccaggaataggcc

SEQ ID NO: 21340 - RNA, 20 nt, synthetic construct
  source 1..20: mol_type = other RNA
tattcctggtaccaggtgag

SEQ ID NO: 21341 - RNA, 20 nt, synthetic construct
  source 1..20: mol_type = other RNA
attcctggtaccaggtgagt

SEQ ID NO: 21342 - RNA, 20 nt, synthetic construct
  source 1..20: mol_type = other RNA
ttcctggtaccaggtgagtg

SEQ ID NO: 21343 - RNA, 20 nt, synthetic construct
  source 1..20: mol_type = other RNA
actcacctggtaccaggaat

SEQ ID NO: 21344 - RNA, 20 nt, synthetic construct
  source 1..20: mol_type = other RNA
tggtaccaggtgagtggggc

SEQ ID NO: 21345 - RNA, 20 nt, synthetic construct
  source 1..20: mol_type = other RNA
ggtaccaggtgagtggggct

SEQ ID NO: 21346 - RNA, 20 nt, synthetic construct
  source 1..20: mol_type = other RNA
gtaccaggtgagtggggctg

SEQ ID NO: 21347 - RNA, 20 nt, synthetic construct
  source 1..20: mol_type = other RNA
agccccactcacctggtacc

SEQ ID NO: 21348 - RNA, 20 nt, synthetic construct
  source 1..20: mol_type = other RNA
ccaggtgagtggggctgggg

SEQ ID NO: 21349 - RNA, 20 nt, synthetic construct
  source 1..20: mol_type = other RNA
ccaccccagccccactcacc

SEQ ID NO: 21350 - RNA, 20 nt, synthetic construct
  source 1..20: mol_type = other RNA
ctggggtggagtccctgtgt

SEQ ID NO: 21351 - RNA, 20 nt, synthetic construct
  source 1..20: mol_type = other RNA
tggggtggagtccctgtgtc

SEQ ID NO: 21352 - RNA, 20 nt, synthetic construct
  source 1..20: mol_type = other RNA
agtccctgtgtcgggaacac

SEQ ID NO: 21353 - RNA, 20 nt, synthetic construct
  source 1..20: mol_type = other RNA
gtccctgtgtcgggaacaca

SEQ ID NO: 21354 - RNA, 20 nt, synthetic construct
  source 1..20: mol_type = other RNA
agccctgtgttcccgacaca

SEQ ID NO: 21355 - RNA, 20 nt, synthetic construct
  source 1..20: mol_type = other RNA
gagccctgtgttcccgacac

SEQ ID NO: 21356 - RNA, 20 nt, synthetic construct
  source 1..20: mol_type = other RNA
gtgagtaactgagtgtcaga

SEQ ID NO: 21357 - RNA, 20 nt, synthetic construct
  source 1..20: mol_type = other RNA
ctgtgtgccagccctgagcc

SEQ ID NO: 21358 - RNA, 20 nt, synthetic construct
  source 1..20: mol_type = other RNA
gctcagggctggcacacagt

SEQ ID NO: 21359 - RNA, 20 nt, synthetic construct
  source 1..20: mol_type = other RNA
agagctcctgggtccagctg

SEQ ID NO: 21360 - RNA, 20 nt, synthetic construct
  source 1..20: mol_type = other RNA
cagctggacccaggagctct

SEQ ID NO: 21361 - RNA, 20 nt, synthetic construct
  source 1..20: mol_type = other RNA
tcagctggacccaggagctc

SEQ ID NO: 21362 - RNA, 20 nt, synthetic construct
  source 1..20: mol_type = other RNA
gggtccagctgaggatcttc

SEQ ID NO: 21363 - RNA, 20 nt, synthetic construct
  source 1..20: mol_type = other RNA
gaagatcctcagctggaccc

SEQ ID NO: 21364 - RNA, 20 nt, synthetic construct
  source 1..20: mol_type = other RNA
gtggccagaagatcctcagc

SEQ ID NO: 21365 - RNA, 20 nt, synthetic construct
  source 1..20: mol_type = other RNA
aggatcttctggccaccttg

SEQ ID NO: 21366 - RNA, 20 nt, synthetic construct
  source 1..20: mol_type = other RNA
ggatcttctggccaccttgc

SEQ ID NO: 21367 - RNA, 20 nt, synthetic construct
  source 1..20: mol_type = other RNA
agggacagcagcccgcaagg

SEQ ID NO: 21368 - RNA, 20 nt, synthetic construct
  source 1..20: mol_type = other RNA
tgcgggctgctgtccctctc

SEQ ID NO: 21369 - RNA, 20 nt, synthetic construct
  source 1..20: mol_type = other RNA
gagagggacagcagcccgca

SEQ ID NO: 21370 - RNA, 20 nt, synthetic construct
  source 1..20: mol_type = other RNA
acaaaggaagtggcctgaga

SEQ ID NO: 21371 - RNA, 20 nt, synthetic construct
  source 1..20: mol_type = other RNA
cacaaaggaagtggcctgag

SEQ ID NO: 21372 - RNA, 20 nt, synthetic construct
  source 1..20: mol_type = other RNA
cttcctttgtgtcctccaag

SEQ ID NO: 21373 - RNA, 20 nt, synthetic construct
  source 1..20: mol_type = other RNA
cttggaggacacaaaggaag

SEQ ID NO: 21374 - RNA, 20 nt, synthetic construct
  source 1..20: mol_type = other RNA
atgccacttggaggacacaa

SEQ ID NO: 21375 - RNA, 20 nt, synthetic construct
  source 1..20: mol_type = other RNA
agggtcagcatgccacttgg

SEQ ID NO: 21376 - RNA, 20 nt, synthetic construct
  source 1..20: mol_type = other RNA
aagagggtcagcatgccact

SEQ ID NO: 21377 - RNA, 20 nt, synthetic construct
  source 1..20: mol_type = other RNA
gtgctgcaggcaaggaaaga

SEQ ID NO: 21378 - RNA, 20 nt, synthetic construct
  source 1..20: mol_type = other RNA
ggtgctgcaggcaaggaaag

SEQ ID NO: 21379 - RNA, 20 nt, synthetic construct
  source 1..20: mol_type = other RNA
gctcgctggtgctgcaggca

SEQ ID NO: 21380 - RNA, 20 nt, synthetic construct
  source 1..20: mol_type = other RNA
catgggctcgctggtgctgc

SEQ ID NO: 21381 - RNA, 20 nt, synthetic construct
  source 1..20: mol_type = other RNA
gcgagcccatgacgacccag

SEQ ID NO: 21382 - RNA, 20 nt, synthetic construct
  source 1..20: mol_type = other RNA
ctgggtcgtcatgggctcgc

SEQ ID NO: 21383 - RNA, 20 nt, synthetic construct
  source 1..20: mol_type = other RNA
tagggccactgggtcgtcat

SEQ ID NO: 21384 - RNA, 20 nt, synthetic construct
  source 1..20: mol_type = other RNA
ttagggccactgggtcgtca

SEQ ID NO: 21385 - RNA, 20 nt, synthetic construct
  source 1..20: mol_type = other RNA
aggtgtactttagggccact

SEQ ID NO: 21386 - RNA, 20 nt, synthetic construct
  source 1..20: mol_type = other RNA
aaggtgtactttagggccac

SEQ ID NO: 21387 - RNA, 20 nt, synthetic construct
  source 1..20: mol_type = other RNA
cctaaagtacaccttccatg

SEQ ID NO: 21388 - RNA, 20 nt, synthetic construct
  source 1..20: mol_type = other RNA
ctcatggaaggtgtacttta

SEQ ID NO: 21389 - RNA, 20 nt, synthetic construct
  source 1..20: mol_type = other RNA
cctcatggaaggtgtacttt

SEQ ID NO: 21390 - RNA, 20 nt, synthetic construct
  source 1..20: mol_type = other RNA
ttccatgaggtgattaccgc

SEQ ID NO: 21391 - RNA, 20 nt, synthetic construct
  source 1..20: mol_type = other RNA
ggcggtaatcacctcatgga

SEQ ID NO: 21392 - RNA, 20 nt, synthetic construct
  source 1..20: mol_type = other RNA
agccggcggtaatcacctca

SEQ ID NO: 21393 - RNA, 20 nt, synthetic construct
  source 1..20: mol_type = other RNA
cgaggatgcgtcagagccgg

SEQ ID NO: 21394 - RNA, 20 nt, synthetic construct
  source 1..20: mol_type = other RNA
cttcgaggatgcgtcagagc

SEQ ID NO: 21395 - RNA, 20 nt, synthetic construct
  source 1..20: mol_type = other RNA
ctggagggcacgcagcttcg

SEQ ID NO: 21396 - RNA, 20 nt, synthetic construct
  source 1..20: mol_type = other RNA
tgccctccagaaccgctgcc

SEQ ID NO: 21397 - RNA, 20 nt, synthetic construct
  source 1..20: mol_type = other RNA
gaccaggcagcggttctgga

SEQ ID NO: 21398 - RNA, 20 nt, synthetic construct
  source 1..20: mol_type = other RNA
ggaccaggcagcggttctgg

SEQ ID NO: 21399 - RNA, 20 nt, synthetic construct
  source 1..20: mol_type = other RNA
accgctgcctggtccctggc

SEQ ID NO: 21400 - RNA, 20 nt, synthetic construct
  source 1..20: mol_type = other RNA
accagccagggaccaggcag

SEQ ID NO: 21401 - RNA, 20 nt, synthetic construct
  source 1..20: mol_type = other RNA
tggcgtaccagccagggacc

SEQ ID NO: 21402 - RNA, 20 nt, synthetic construct
  source 1..20: mol_type = other RNA
tgtgggtggcgtaccagcca

SEQ ID NO: 21403 - RNA, 20 nt, synthetic construct
  source 1..20: mol_type = other RNA
atgtgggtggcgtaccagcc

SEQ ID NO: 21404 - RNA, 20 nt, synthetic construct
  source 1..20: mol_type = other RNA
acgccacccacatcgagcgc

SEQ ID NO: 21405 - RNA, 20 nt, synthetic construct
  source 1..20: mol_type = other RNA
gagccagcgctcgatgtggg

SEQ ID NO: 21406 - RNA, 20 nt, synthetic construct
  source 1..20: mol_type = other RNA
actgagccagcgctcgatgt

SEQ ID NO: 21407 - RNA, 20 nt, synthetic construct
  source 1..20: mol_type = other RNA
cactgagccagcgctcgatg

SEQ ID NO: 21408 - RNA, 20 nt, synthetic construct
  source 1..20: mol_type = other RNA
cagtgcctatcacgccaacc

SEQ ID NO: 21409 - RNA, 20 nt, synthetic construct
  source 1..20: mol_type = other RNA
agctacctggttggcgtgat

SEQ ID NO: 21410 - RNA, 20 nt, synthetic construct
  source 1..20: mol_type = other RNA
agggacagcagctacctggt

SEQ ID NO: 21411 - RNA, 20 nt, synthetic construct
  source 1..20: mol_type = other RNA
ggtcagggacagcagctacc

SEQ ID NO: 21412 - RNA, 20 nt, synthetic construct
  source 1..20: mol_type = other RNA
tgctgtccctgacccttgtg

SEQ ID NO: 21413 - RNA, 20 nt, synthetic construct
  source 1..20: mol_type = other RNA
gctgtccctgacccttgtga

SEQ ID NO: 21414 - RNA, 20 nt, synthetic construct
  source 1..20: mol_type = other RNA
gactgccctcacaagggtca

SEQ ID NO: 21415 - RNA, 20 nt, synthetic construct
  source 1..20: mol_type = other RNA
tgactgccctcacaagggtc

SEQ ID NO: 21416 - RNA, 20 nt, synthetic construct
  source 1..20: mol_type = other RNA
tgtgagggcagtcacagtac

SEQ ID NO: 21417 - RNA, 20 nt, synthetic construct
  source 1..20: mol_type = other RNA
tactgtgactgccctcacaa

SEQ ID NO: 21418 - RNA, 20 nt, synthetic construct
  source 1..20: mol_type = other RNA
gtactgtgactgccctcaca

SEQ ID NO: 21419 - RNA, 20 nt, synthetic construct
  source 1..20: mol_type = other RNA
gtcacagtactggcttgctg

SEQ ID NO: 21420 - RNA, 20 nt, synthetic construct
  source 1..20: mol_type = other RNA
tactggcttgctgtggttag

SEQ ID NO: 21421 - RNA, 20 nt, synthetic construct
  source 1..20: mol_type = other RNA
caactctttctcaccagccg

SEQ ID NO: 21422 - RNA, 20 nt, synthetic construct
  source 1..20: mol_type = other RNA
ggctggtgagaaagagttgg

SEQ ID NO: 21423 - RNA, 20 nt, synthetic construct
  source 1..20: mol_type = other RNA
actctttctcaccagccgtg

SEQ ID NO: 21424 - RNA, 20 nt, synthetic construct
  source 1..20: mol_type = other RNA
cacggctggtgagaaagagt

SEQ ID NO: 21425 - RNA, 20 nt, synthetic construct
  source 1..20: mol_type = other RNA
ggcatatctgtccccacggc

SEQ ID NO: 21426 - RNA, 20 nt, synthetic construct
  source 1..20: mol_type = other RNA
ggggacagatatgccctcct

SEQ ID NO: 21427 - RNA, 20 nt, synthetic construct
  source 1..20: mol_type = other RNA
ggagggcatatctgtcccca

SEQ ID NO: 21428 - RNA, 20 nt, synthetic construct
  source 1..20: mol_type = other RNA
agccagttctagagggtgca

SEQ ID NO: 21429 - RNA, 20 nt, synthetic construct
  source 1..20: mol_type = other RNA
gaccctgcaccctctagaac

SEQ ID NO: 21430 - RNA, 20 nt, synthetic construct
  source 1..20: mol_type = other RNA
agggtcccatatttataagc

SEQ ID NO: 21431 - RNA, 20 nt, synthetic construct
  source 1..20: mol_type = other RNA
atgggcctgcttataaatat

SEQ ID NO: 21432 - RNA, 20 nt, synthetic construct
  source 1..20: mol_type = other RNA
aatgggcctgcttataaata

SEQ ID NO: 21433 - RNA, 20 nt, synthetic construct
  source 1..20: mol_type = other RNA
caggcccattcctgctgccg

SEQ ID NO: 21434 - RNA, 20 nt, synthetic construct
  source 1..20: mol_type = other RNA
acagccacggcagcaggaat

SEQ ID NO: 21435 - RNA, 20 nt, synthetic construct
  source 1..20: mol_type = other RNA
aacagccacggcagcaggaa

SEQ ID NO: 21436 - RNA, 20 nt, synthetic construct
  source 1..20: mol_type = other RNA
agggcaacagccacggcagc

SEQ ID NO: 21437 - RNA, 20 nt, synthetic construct
  source 1..20: mol_type = other RNA
gcaaacaagggcaacagcca

SEQ ID NO: 21438 - RNA, 20 nt, synthetic construct
  source 1..20: mol_type = other RNA
ttgacttcggtggcaaacaa

SEQ ID NO: 21439 - RNA, 20 nt, synthetic construct
  source 1..20: mol_type = other RNA
tttgccaccgaagtcaaagc

SEQ ID NO: 21440 - RNA, 20 nt, synthetic construct
  source 1..20: mol_type = other RNA
gggacctgctttgacttcgg

SEQ ID NO: 21441 - RNA, 20 nt, synthetic construct
  source 1..20: mol_type = other RNA
atcgggacctgctttgactt

SEQ ID NO: 21442 - RNA, 20 nt, synthetic construct
  source 1..20: mol_type = other RNA
ggaaagggagaaaggggatc

SEQ ID NO: 21443 - RNA, 20 nt, synthetic construct
  source 1..20: mol_type = other RNA
tggaaagggagaaaggggat

SEQ ID NO: 21444 - RNA, 20 nt, synthetic construct
  source 1..20: mol_type = other RNA
ctttctccctttccagattc

SEQ ID NO: 21445 - RNA, 20 nt, synthetic construct
  source 1..20: mol_type = other RNA
gaatctggaaagggagaaag

SEQ ID NO: 21446 - RNA, 20 nt, synthetic construct
  source 1..20: mol_type = other RNA
agaatctggaaagggagaaa

SEQ ID NO: 21447 - RNA, 20 nt, synthetic construct
  source 1..20: mol_type = other RNA
cagaatctggaaagggagaa

SEQ ID NO: 21448 - RNA, 20 nt, synthetic construct
  source 1..20: mol_type = other RNA
ccctttccagattctggtct

SEQ ID NO: 21449 - RNA, 20 nt, synthetic construct
  source 1..20: mol_type = other RNA
ttccagattctggtcttgga

SEQ ID NO: 21450 - RNA, 20 nt, synthetic construct
  source 1..20: mol_type = other RNA
ccaagaccagaatctggaaa

SEQ ID NO: 21451 - RNA, 20 nt, synthetic construct
  source 1..20: mol_type = other RNA
tccaagaccagaatctggaa

SEQ ID NO: 21452 - RNA, 20 nt, synthetic construct
  source 1..20: mol_type = other RNA
tgccatccaagaccagaatc

SEQ ID NO: 21453 - RNA, 20 nt, synthetic construct
  source 1..20: mol_type = other RNA
cacagaacctgccaaagtga

SEQ ID NO: 21454 - RNA, 20 nt, synthetic construct
  source 1..20: mol_type = other RNA
acctgccaaagtgatggaca

SEQ ID NO: 21455 - RNA, 20 nt, synthetic construct
  source 1..20: mol_type = other RNA
accatgtccatcactttggc

SEQ ID NO: 21456 - RNA, 20 nt, synthetic construct
  source 1..20: mol_type = other RNA
ctgcaccatgtccatcactt

SEQ ID NO: 21457 - RNA, 20 nt, synthetic construct
  source 1..20: mol_type = other RNA
gacatggtgcagaagttcct

SEQ ID NO: 21458 - RNA, 20 nt, synthetic construct
  source 1..20: mol_type = other RNA
acatggtgcagaagttcctt

SEQ ID NO: 21459 - RNA, 20 nt, synthetic construct
  source 1..20: mol_type = other RNA
catggtgcagaagttccttg

SEQ ID NO: 21460 - RNA, 20 nt, synthetic construct
  source 1..20: mol_type = other RNA
caatggtgttggtcacccca

SEQ ID NO: 21461 - RNA, 20 nt, synthetic construct
  source 1..20: mol_type = other RNA
tttgtggtagtcaatggtgt

SEQ ID NO: 21462 - RNA, 20 nt, synthetic construct
  source 1..20: mol_type = other RNA
cattgactaccacaaaacct

SEQ ID NO: 21463 - RNA, 20 nt, synthetic construct
  source 1..20: mol_type = other RNA
caaggttttgtggtagtcaa

SEQ ID NO: 21464 - RNA, 20 nt, synthetic construct
  source 1..20: mol_type = other RNA
acactcacgccaaggttttg

SEQ ID NO: 21465 - RNA, 20 nt, synthetic construct
  source 1..20: mol_type = other RNA
aaaaggcaacactcacgcca

SEQ ID NO: 21466 - RNA, 20 nt, synthetic construct
  source 1..20: mol_type = other RNA
tgttgccttttcctttctgc

SEQ ID NO: 21467 - RNA, 20 nt, synthetic construct
  source 1..20: mol_type = other RNA
aataacctgcagaaaggaaa

SEQ ID NO: 21468 - RNA, 20 nt, synthetic construct
  source 1..20: mol_type = other RNA
cagggaaataacctgcagaa

SEQ ID NO: 21469 - RNA, 20 nt, synthetic construct
  source 1..20: mol_type = other RNA
tgcaggttatttccctgata

SEQ ID NO: 21470 - RNA, 20 nt, synthetic construct
  source 1..20: mol_type = other RNA
tatttccctgataaggcacc

SEQ ID NO: 21471 - RNA, 20 nt, synthetic construct
  source 1..20: mol_type = other RNA
atttccctgataaggcacct

SEQ ID NO: 21472 - RNA, 20 nt, synthetic construct
  source 1..20: mol_type = other RNA
ttggcccaggtgccttatca

SEQ ID NO: 21473 - RNA, 20 nt, synthetic construct
  source 1..20: mol_type = other RNA
gttggcccaggtgccttatc

SEQ ID NO: 21474 - RNA, 20 nt, synthetic construct
  source 1..20: mol_type = other RNA
gactttggctttgttggccc

SEQ ID NO: 21475 - RNA, 20 nt, synthetic construct
  source 1..20: mol_type = other RNA
attcaagactttggctttgt

SEQ ID NO: 21476 - RNA, 20 nt, synthetic construct
  source 1..20: mol_type = other RNA
ctcataattattcaagactt

SEQ ID NO: 21477 - RNA, 20 nt, synthetic construct
  source 1..20: mol_type = other RNA
ttagttagagtcagaaagta

SEQ ID NO: 21478 - RNA, 20 nt, synthetic construct
  source 1..20: mol_type = other RNA
ctactgctcttgaacccaca

SEQ ID NO: 21479 - RNA, 20 nt, synthetic construct
  source 1..20: mol_type = other RNA
ttcaagagcagtagattccc

SEQ ID NO: 21480 - RNA, 20 nt, synthetic construct
  source 1..20: mol_type = other RNA
tccctggtctctgccattcc

SEQ ID NO: 21481 - RNA, 20 nt, synthetic construct
  source 1..20: mol_type = other RNA
ccctggtctctgccattcct

SEQ ID NO: 21482 - RNA, 20 nt, synthetic construct
  source 1..20: mol_type = other RNA
cctggtctctgccattcctg

SEQ ID NO: 21483 - RNA, 20 nt, synthetic construct
  source 1..20: mol_type = other RNA
cccaggaatggcagagacca

SEQ ID NO: 21484 - RNA, 20 nt, synthetic construct
  source 1..20: mol_type = other RNA
ccccaggaatggcagagacc

SEQ ID NO: 21485 - RNA, 20 nt, synthetic construct
  source 1..20: mol_type = other RNA
attcctggggtccatgaaca

SEQ ID NO: 21486 - RNA, 20 nt, synthetic construct
  source 1..20: mol_type = other RNA
atgttcatggaccccaggaa

SEQ ID NO: 21487 - RNA, 20 nt, synthetic construct
  source 1..20: mol_type = other RNA
ggtccatgaacatggcttta

SEQ ID NO: 21488 - RNA, 20 nt, synthetic construct
  source 1..20: mol_type = other RNA
catgaacatggctttaaggt

SEQ ID NO: 21489 - RNA, 20 nt, synthetic construct
  source 1..20: mol_type = other RNA
cgaccttaaagccatgttca

SEQ ID NO: 21490 - RNA, 20 nt, synthetic construct
  source 1..20: mol_type = other RNA
catggctttaaggtcggaag

SEQ ID NO: 21491 - RNA, 20 nt, synthetic construct
  source 1..20: mol_type = other RNA
atggctttaaggtcggaagt

SEQ ID NO: 21492 - RNA, 20 nt, synthetic construct
  source 1..20: mol_type = other RNA
gctttaaggtcggaagtggg

SEQ ID NO: 21493 - RNA, 20 nt, synthetic construct
  source 1..20: mol_type = other RNA
gaaagtctttggatgggagc

SEQ ID NO: 21494 - RNA, 20 nt, synthetic construct
  source 1..20: mol_type = other RNA
aggtgggaaagtctttggat

SEQ ID NO: 21495 - RNA, 20 nt, synthetic construct
  source 1..20: mol_type = other RNA
gaggtgggaaagtctttgga

SEQ ID NO: 21496 - RNA, 20 nt, synthetic construct
  source 1..20: mol_type = other RNA
aaagactttcccacctccac

SEQ ID NO: 21497 - RNA, 20 nt, synthetic construct
  source 1..20: mol_type = other RNA
tgtggaggtgggaaagtctt

SEQ ID NO: 21498 - RNA, 20 nt, synthetic construct
  source 1..20: mol_type = other RNA
tggatcaaacctgtggaggt

SEQ ID NO: 21499 - RNA, 20 nt, synthetic construct
  source 1..20: mol_type = other RNA
ttggatcaaacctgtggagg

SEQ ID NO: 21500 - RNA, 20 nt, synthetic construct
  source 1..20: mol_type = other RNA
cacaggtttgatccaaagaa

SEQ ID NO: 21501 - RNA, 20 nt, synthetic construct
  source 1..20: mol_type = other RNA
tctttggatcaaacctgtgg

SEQ ID NO: 21502 - RNA, 20 nt, synthetic construct
  source 1..20: mol_type = other RNA
ctttctttggatcaaacctg

SEQ ID NO: 21503 - RNA, 20 nt, synthetic construct
  source 1..20: mol_type = other RNA
ttgatccaaagaaaggattt

SEQ ID NO: 21504 - RNA, 20 nt, synthetic construct
  source 1..20: mol_type = other RNA
tggcaccaaaatcctttctt

SEQ ID NO: 21505 - RNA, 20 nt, synthetic construct
  source 1..20: mol_type = other RNA
ttttggtgccaactgcttga

SEQ ID NO: 21506 - RNA, 20 nt, synthetic construct
  source 1..20: mol_type = other RNA
tggtgccaactgcttgaagg

SEQ ID NO: 21507 - RNA, 20 nt, synthetic construct
  source 1..20: mol_type = other RNA
tttttcctccttcaagcagt

SEQ ID NO: 21508 - RNA, 20 nt, synthetic construct
  source 1..20: mol_type = other RNA
aggaggaaaaaccaagtgtc

SEQ ID NO: 21509 - RNA, 20 nt, synthetic construct
  source 1..20: mol_type = other RNA
ggaggaaaaaccaagtgtct

SEQ ID NO: 21510 - RNA, 20 nt, synthetic construct
  source 1..20: mol_type = other RNA
caagtgtctgggcaaaagca

SEQ ID NO: 21511 - RNA, 20 nt, synthetic construct
  source 1..20: mol_type = other RNA
aagtgtctgggcaaaagcaa

SEQ ID NO: 21512 - RNA, 20 nt, synthetic construct
  source 1..20: mol_type = other RNA
cttgcttttgcccagacact

SEQ ID NO: 21513 - RNA, 20 nt, synthetic construct
  source 1..20: mol_type = other RNA
gtctgggcaaaagcaagggc

SEQ ID NO: 21514 - RNA, 20 nt, synthetic construct
  source 1..20: mol_type = other RNA
gggccggaaatatcccgaga

SEQ ID NO: 21515 - RNA, 20 nt, synthetic construct
  source 1..20: mol_type = other RNA
gaaatatcccgagatggact

SEQ ID NO: 21516 - RNA, 20 nt, synthetic construct
  source 1..20: mol_type = other RNA
agtccatctcgggatatttc

SEQ ID NO: 21517 - RNA, 20 nt, synthetic construct
  source 1..20: mol_type = other RNA
gagatggacttggatgtaag

SEQ ID NO: 21518 - RNA, 20 nt, synthetic construct
  source 1..20: mol_type = other RNA
cttacatccaagtccatctc

SEQ ID NO: 21519 - RNA, 20 nt, synthetic construct
  source 1..20: mol_type = other RNA
acttacatccaagtccatct

SEQ ID NO: 21520 - RNA, 20 nt, synthetic construct
  source 1..20: mol_type = other RNA
ctacctgtagcacctgcata

SEQ ID NO: 21521 - RNA, 20 nt, synthetic construct
  source 1..20: mol_type = other RNA
tacctgtagcacctgcataa

SEQ ID NO: 21522 - RNA, 20 nt, synthetic construct
  source 1..20: mol_type = other RNA
gtagcacctgcataagggta

SEQ ID NO: 21523 - RNA, 20 nt, synthetic construct
  source 1..20: mol_type = other RNA
tagcacctgcataagggtaa

SEQ ID NO: 21524 - RNA, 20 nt, synthetic construct
  source 1..20: mol_type = other RNA
tacccttatgcaggtgctac

SEQ ID NO: 21525 - RNA, 20 nt, synthetic construct
  source 1..20: mol_type = other RNA
gggaccccttacccttatgc

SEQ ID NO: 21526 - RNA, 20 nt, synthetic construct
  source 1..20: mol_type = other RNA
aagggtaaggggtccctgta

SEQ ID NO: 21527 - RNA, 20 nt, synthetic construct
  source 1..20: mol_type = other RNA
ggggtccctgtatggagttg

SEQ ID NO: 21528 - RNA, 20 nt, synthetic construct
  source 1..20: mol_type = other RNA
gggtccctgtatggagttga

SEQ ID NO: 21529 - RNA, 20 nt, synthetic construct
  source 1..20: mol_type = other RNA
ggtccctgtatggagttgag

SEQ ID NO: 21530 - RNA, 20 nt, synthetic construct
  source 1..20: mol_type = other RNA
gtccctgtatggagttgagg

SEQ ID NO: 21531 - RNA, 20 nt, synthetic construct
  source 1..20: mol_type = other RNA
atccccctcaactccataca

SEQ ID NO: 21532 - RNA, 20 nt, synthetic construct
  source 1..20: mol_type = other RNA
aatccccctcaactccatac

SEQ ID NO: 21533 - RNA, 20 nt, synthetic construct
  source 1..20: mol_type = other RNA
acatgctgagtgcatggtaa

SEQ ID NO: 21534 - RNA, 20 nt, synthetic construct
  source 1..20: mol_type = other RNA
ccatgcactcagcatgttca

SEQ ID NO: 21535 - RNA, 20 nt, synthetic construct
  source 1..20: mol_type = other RNA
ccatgaacatgctgagtgca

SEQ ID NO: 21536 - RNA, 20 nt, synthetic construct
  source 1..20: mol_type = other RNA
ttcatggccttagcatttct

SEQ ID NO: 21537 - RNA, 20 nt, synthetic construct
  source 1..20: mol_type = other RNA
cccagcactttgggaggccg

SEQ ID NO: 21538 - RNA, 20 nt, synthetic construct
  source 1..20: mol_type = other RNA
tcccaaagtgctgggattac

SEQ ID NO: 21539 - RNA, 20 nt, synthetic construct
  source 1..20: mol_type = other RNA
tgtaatcccagcactttggg

SEQ ID NO: 21540 - RNA, 20 nt, synthetic construct
  source 1..20: mol_type = other RNA
gcctgtaatcccagcacttt

SEQ ID NO: 21541 - RNA, 20 nt, synthetic construct
  source 1..20: mol_type = other RNA
tgcctgtaatcccagcactt

SEQ ID NO: 21542 - RNA, 20 nt, synthetic construct
  source 1..20: mol_type = other RNA
caggcatgagccaccgtgcc

SEQ ID NO: 21543 - RNA, 20 nt, synthetic construct
  source 1..20: mol_type = other RNA
ccaccgtgcccggccgagca

SEQ ID NO: 21544 - RNA, 20 nt, synthetic construct
  source 1..20: mol_type = other RNA
ccatgctcggccgggcacgg

SEQ ID NO: 21545 - RNA, 20 nt, synthetic construct
  source 1..20: mol_type = other RNA
tcgccatgctcggccgggca

SEQ ID NO: 21546 - RNA, 20 nt, synthetic construct
  source 1..20: mol_type = other RNA
aaaaatcgccatgctcggcc

SEQ ID NO: 21547 - RNA, 20 nt, synthetic construct
  source 1..20: mol_type = other RNA
taaaaatcgccatgctcggc

SEQ ID NO: 21548 - RNA, 20 nt, synthetic construct
  source 1..20: mol_type = other RNA
agcatggcgatttttagagg

SEQ ID NO: 21549 - RNA, 20 nt, synthetic construct
  source 1..20: mol_type = other RNA
cctctaaaaatcgccatgct

SEQ ID NO: 21550 - RNA, 20 nt, synthetic construct
  source 1..20: mol_type = other RNA
cactcttaagtcagtacaca

SEQ ID NO: 21551 - RNA, 20 nt, synthetic construct
  source 1..20: mol_type = other RNA
ggctcgggactgtaacggga

SEQ ID NO: 21552 - RNA, 20 nt, synthetic construct
  source 1..20: mol_type = other RNA
ggaaggctcgggactgtaac

SEQ ID NO: 21553 - RNA, 20 nt, synthetic construct
  source 1..20: mol_type = other RNA
aggaaggctcgggactgtaa

SEQ ID NO: 21554 - RNA, 20 nt, synthetic construct
  source 1..20: mol_type = other RNA
atagtccttcaggaaggctc

SEQ ID NO: 21555 - RNA, 20 nt, synthetic construct
  source 1..20: mol_type = other RNA
aatagtccttcaggaaggct

SEQ ID NO: 21556 - RNA, 20 nt, synthetic construct
  source 1..20: mol_type = other RNA
cttcctgaaggactattacc

SEQ ID NO: 21557 - RNA, 20 nt, synthetic construct
  source 1..20: mol_type = other RNA
ccggtaatagtccttcagga

SEQ ID NO: 21558 - RNA, 20 nt, synthetic construct
  source 1..20: mol_type = other RNA
ggtcccggtaatagtccttc

SEQ ID NO: 21559 - RNA, 20 nt, synthetic construct
  source 1..20: mol_type = other RNA
agagctcgatgttgtggtcc

SEQ ID NO: 21560 - RNA, 20 nt, synthetic construct
  source 1..20: mol_type = other RNA
gcttggagagctcgatgttg

SEQ ID NO: 21561 - RNA, 20 nt, synthetic construct
  source 1..20: mol_type = other RNA
ctccaagctgctgtataaga

SEQ ID NO: 21562 - RNA, 20 nt, synthetic construct
  source 1..20: mol_type = other RNA
tccaagctgctgtataagat

SEQ ID NO: 21563 - RNA, 20 nt, synthetic construct
  source 1..20: mol_type = other RNA
gcccatcttatacagcagct

SEQ ID NO: 21564 - RNA, 20 nt, synthetic construct
  source 1..20: mol_type = other RNA
tgggccagacacttcccact

SEQ ID NO: 21565 - RNA, 20 nt, synthetic construct
  source 1..20: mol_type = other RNA
gtagccaagtgggaagtgtc

SEQ ID NO: 21566 - RNA, 20 nt, synthetic construct
  source 1..20: mol_type = other RNA
acttcccacttggctacgag

SEQ ID NO: 21567 - RNA, 20 nt, synthetic construct
  source 1..20: mol_type = other RNA
aggtcctctcgtagccaagt

SEQ ID NO: 21568 - RNA, 20 nt, synthetic construct
  source 1..20: mol_type = other RNA
gaggtcctctcgtagccaag

SEQ ID NO: 21569 - RNA, 20 nt, synthetic construct
  source 1..20: mol_type = other RNA
gagaggacctccagaacacc

SEQ ID NO: 21570 - RNA, 20 nt, synthetic construct
  source 1..20: mol_type = other RNA
tccagaacaccaggtagccg

SEQ ID NO: 21571 - RNA, 20 nt, synthetic construct
  source 1..20: mol_type = other RNA
acggctacctggtgttctgg

SEQ ID NO: 21572 - RNA, 20 nt, synthetic construct
  source 1..20: mol_type = other RNA
gccacggctacctggtgttc

SEQ ID NO: 21573 - RNA, 20 nt, synthetic construct
  source 1..20: mol_type = other RNA
ctgtggtggccacggctacc

SEQ ID NO: 21574 - RNA, 20 nt, synthetic construct
  source 1..20: mol_type = other RNA
cagtctggctgtggtggcca

SEQ ID NO: 21575 - RNA, 20 nt, synthetic construct
  source 1..20: mol_type = other RNA
aacgttcagtctggctgtgg

SEQ ID NO: 21576 - RNA, 20 nt, synthetic construct
  source 1..20: mol_type = other RNA
acaaacgttcagtctggctg

SEQ ID NO: 21577 - RNA, 20 nt, synthetic construct
  source 1..20: mol_type = other RNA
gactgaacgtttgtgaaagc

SEQ ID NO: 21578 - RNA, 20 nt, synthetic construct
  source 1..20: mol_type = other RNA
actgaacgtttgtgaaagct

SEQ ID NO: 21579 - RNA, 20 nt, synthetic construct
  source 1..20: mol_type = other RNA
gctttcacaaacgttcagtc

SEQ ID NO: 21580 - RNA, 20 nt, synthetic construct
  source 1..20: mol_type = other RNA
ggtctggctcagcgtgtggt

SEQ ID NO: 21581 - RNA, 20 nt, synthetic construct
  source 1..20: mol_type = other RNA
aggtctggctcagcgtgtgg

SEQ ID NO: 21582 - RNA, 20 nt, synthetic construct
  source 1..20: mol_type = other RNA
tgcaggtctggctcagcgtg

SEQ ID NO: 21583 - RNA, 20 nt, synthetic construct
  source 1..20: mol_type = other RNA
gctgagccagacctgcagag

SEQ ID NO: 21584 - RNA, 20 nt, synthetic construct
  source 1..20: mol_type = other RNA
ctgagccagacctgcagagt

SEQ ID NO: 21585 - RNA, 20 nt, synthetic construct
  source 1..20: mol_type = other RNA
agacctgcagagtgggaagc

SEQ ID NO: 21586 - RNA, 20 nt, synthetic construct
  source 1..20: mol_type = other RNA
agcttcccactctgcaggtc

SEQ ID NO: 21587 - RNA, 20 nt, synthetic construct
  source 1..20: mol_type = other RNA
gcagagtgggaagctggacc

SEQ ID NO: 21588 - RNA, 20 nt, synthetic construct
  source 1..20: mol_type = other RNA
cagagtgggaagctggacca

SEQ ID NO: 21589 - RNA, 20 nt, synthetic construct
  source 1..20: mol_type = other RNA
ggtccagcttcccactctgc

SEQ ID NO: 21590 - RNA, 20 nt, synthetic construct
  source 1..20: mol_type = other RNA
tcataagtgcgcagctgccc

SEQ ID NO: 21591 - RNA, 20 nt, synthetic construct
  source 1..20: mol_type = other RNA
cacttatgagcaatactctg

SEQ ID NO: 21592 - RNA, 20 nt, synthetic construct
  source 1..20: mol_type = other RNA
ttatgagcaatactctgtgg

SEQ ID NO: 21593 - RNA, 20 nt, synthetic construct
  source 1..20: mol_type = other RNA
agcaatactctgtggaggtc

SEQ ID NO: 21594 - RNA, 20 nt, synthetic construct
  source 1..20: mol_type = other RNA
aatactctgtggaggtctgg

SEQ ID NO: 21595 - RNA, 20 nt, synthetic construct
  source 1..20: mol_type = other RNA
atactctgtggaggtctggt

SEQ ID NO: 21596 - RNA, 20 nt, synthetic construct
  source 1..20: mol_type = other RNA
tactctgtggaggtctggtg

SEQ ID NO: 21597 - RNA, 20 nt, synthetic construct
  source 1..20: mol_type = other RNA
ctgtggaggtctggtggggc

SEQ ID NO: 21598 - RNA, 20 nt, synthetic construct
  source 1..20: mol_type = other RNA
tgtggaggtctggtggggct

SEQ ID NO: 21599 - RNA, 20 nt, synthetic construct
  source 1..20: mol_type = other RNA
gtggaggtctggtggggctg

SEQ ID NO: 21600 - RNA, 20 nt, synthetic construct
  source 1..20: mol_type = other RNA
tggaggtctggtggggctgg

SEQ ID NO: 21601 - RNA, 20 nt, synthetic construct
  source 1..20: mol_type = other RNA
gtggggctgggggagcaccc

SEQ ID NO: 21602 - RNA, 20 nt, synthetic construct
  source 1..20: mol_type = other RNA
gggctgggggagcacccagg

SEQ ID NO: 21603 - RNA, 20 nt, synthetic construct
  source 1..20: mol_type = other RNA
aggcggatctgcaagcacct

SEQ ID NO: 21604 - RNA, 20 nt, synthetic construct
  source 1..20: mol_type = other RNA
aggtgcttgcagatccgcct

SEQ ID NO: 21605 - RNA, 20 nt, synthetic construct
  source 1..20: mol_type = other RNA
gaggtgcttgcagatccgcc

SEQ ID NO: 21606 - RNA, 20 nt, synthetic construct
  source 1..20: mol_type = other RNA
cacctcggagcacccaccgc

SEQ ID NO: 21607 - RNA, 20 nt, synthetic construct
  source 1..20: mol_type = other RNA
acctcggagcacccaccgct

SEQ ID NO: 21608 - RNA, 20 nt, synthetic construct
  source 1..20: mol_type = other RNA
acccagcggtgggtgctccg

SEQ ID NO: 21609 - RNA, 20 nt, synthetic construct
  source 1..20: mol_type = other RNA
agcacccaccgctgggtctg

SEQ ID NO: 21610 - RNA, 20 nt, synthetic construct
  source 1..20: mol_type = other RNA
accgctgggtctgcggccta

SEQ ID NO: 21611 - RNA, 20 nt, synthetic construct
  source 1..20: mol_type = other RNA
ccgctgggtctgcggcctaa

SEQ ID NO: 21612 - RNA, 20 nt, synthetic construct
  source 1..20: mol_type = other RNA
taggccgcagacccagcggt

SEQ ID NO: 21613 - RNA, 20 nt, synthetic construct
  source 1..20: mol_type = other RNA
ttaggccgcagacccagcgg

SEQ ID NO: 21614 - RNA, 20 nt, synthetic construct
  source 1..20: mol_type = other RNA
cccttaggccgcagacccag

SEQ ID NO: 21615 - RNA, 20 nt, synthetic construct
  source 1..20: mol_type = other RNA
gctggcgagggaggtccctt

SEQ ID NO: 21616 - RNA, 20 nt, synthetic construct
  source 1..20: mol_type = other RNA
tggacctctgctggcgaggg

SEQ ID NO: 21617 - RNA, 20 nt, synthetic construct
  source 1..20: mol_type = other RNA
gaatggacctctgctggcga

SEQ ID NO: 21618 - RNA, 20 nt, synthetic construct
  source 1..20: mol_type = other RNA
ggaatggacctctgctggcg

SEQ ID NO: 21619 - RNA, 20 nt, synthetic construct
  source 1..20: mol_type = other RNA
ggaacggaatggacctctgc

SEQ ID NO: 21620 - RNA, 20 nt, synthetic construct
  source 1..20: mol_type = other RNA
attccgttcccagctgctcc

SEQ ID NO: 21621 - RNA, 20 nt, synthetic construct
  source 1..20: mol_type = other RNA
ttccgttcccagctgctcct

SEQ ID NO: 21622 - RNA, 20 nt, synthetic construct
  source 1..20: mol_type = other RNA
tccgttcccagctgctcctg

SEQ ID NO: 21623 - RNA, 20 nt, synthetic construct
  source 1..20: mol_type = other RNA
aggagcagctgggaacggaa

SEQ ID NO: 21624 - RNA, 20 nt, synthetic construct
  source 1..20: mol_type = other RNA
gttcccagctgctcctgggg

SEQ ID NO: 21625 - RNA, 20 nt, synthetic construct
  source 1..20: mol_type = other RNA
tccccaggagcagctgggaa

SEQ ID NO: 21626 - RNA, 20 nt, synthetic construct
  source 1..20: mol_type = other RNA
cggcctccccaggagcagct

SEQ ID NO: 21627 - RNA, 20 nt, synthetic construct
  source 1..20: mol_type = other RNA
gcggcctccccaggagcagc

SEQ ID NO: 21628 - RNA, 20 nt, synthetic construct
  source 1..20: mol_type = other RNA
ctcctggggaggccgcttcc

SEQ ID NO: 21629 - RNA, 20 nt, synthetic construct
  source 1..20: mol_type = other RNA
tggggaggccgcttcctggt

SEQ ID NO: 21630 - RNA, 20 nt, synthetic construct
  source 1..20: mol_type = other RNA
taccaggaagcggcctcccc

SEQ ID NO: 21631 - RNA, 20 nt, synthetic construct
  source 1..20: mol_type = other RNA
gaggccgcttcctggtagga

SEQ ID NO: 21632 - RNA, 20 nt, synthetic construct
  source 1..20: mol_type = other RNA
gactccctcctaccaggaag

SEQ ID NO: 21633 - RNA, 20 nt, synthetic construct
  source 1..20: mol_type = other RNA
ctcgtggactccctcctacc

SEQ ID NO: 21634 - RNA, 20 nt, synthetic construct
  source 1..20: mol_type = other RNA
agggacagaaaagagtctcg

SEQ ID NO: 21635 - RNA, 20 nt, synthetic construct
  source 1..20: mol_type = other RNA
cagtcggcggaacacagtga

SEQ ID NO: 21636 - RNA, 20 nt, synthetic construct
  source 1..20: mol_type = other RNA
acagtcggcggaacacagtg

SEQ ID NO: 21637 - RNA, 20 nt, synthetic construct
  source 1..20: mol_type = other RNA
tgacgagaggggacagtcgg

SEQ ID NO: 21638 - RNA, 20 nt, synthetic construct
  source 1..20: mol_type = other RNA
gggtgacgagaggggacagt

SEQ ID NO: 21639 - RNA, 20 nt, synthetic construct
  source 1..20: mol_type = other RNA
ggagtgatgggtgacgagag

SEQ ID NO: 21640 - RNA, 20 nt, synthetic construct
  source 1..20: mol_type = other RNA
gggagtgatgggtgacgaga

SEQ ID NO: 21641 - RNA, 20 nt, synthetic construct
  source 1..20: mol_type = other RNA
agggagtgatgggtgacgag

SEQ ID NO: 21642 - RNA, 20 nt, synthetic construct
  source 1..20: mol_type = other RNA
ccatcactccctgcttccgc

SEQ ID NO: 21643 - RNA, 20 nt, synthetic construct
  source 1..20: mol_type = other RNA
catcactccctgcttccgca

SEQ ID NO: 21644 - RNA, 20 nt, synthetic construct
  source 1..20: mol_type = other RNA
ctgcggaagcagggagtgat

SEQ ID NO: 21645 - RNA, 20 nt, synthetic construct
  source 1..20: mol_type = other RNA
cctgcggaagcagggagtga

SEQ ID NO: 21646 - RNA, 20 nt, synthetic construct
  source 1..20: mol_type = other RNA
aggggcgccctgcggaagca

SEQ ID NO: 21647 - RNA, 20 nt, synthetic construct
  source 1..20: mol_type = other RNA
gaggggcgccctgcggaagc

SEQ ID NO: 21648 - RNA, 20 nt, synthetic construct
  source 1..20: mol_type = other RNA
gaatactgaggggcgccctg

SEQ ID NO: 21649 - RNA, 20 nt, synthetic construct
  source 1..20: mol_type = other RNA
atatggcagcgaatactgag

SEQ ID NO: 21650 - RNA, 20 nt, synthetic construct
  source 1..20: mol_type = other RNA
catatggcagcgaatactga

SEQ ID NO: 21651 - RNA, 20 nt, synthetic construct
  source 1..20: mol_type = other RNA
acatatggcagcgaatactg

SEQ ID NO: 21652 - RNA, 20 nt, synthetic construct
  source 1..20: mol_type = other RNA
gccatatgtccctgtcctcc

SEQ ID NO: 21653 - RNA, 20 nt, synthetic construct
  source 1..20: mol_type = other RNA
gcctggaggacagggacata

SEQ ID NO: 21654 - RNA, 20 nt, synthetic construct
  source 1..20: mol_type = other RNA
gtccctgtcctccaggctgt

SEQ ID NO: 21655 - RNA, 20 nt, synthetic construct
  source 1..20: mol_type = other RNA
tccctgtcctccaggctgta

SEQ ID NO: 21656 - RNA, 20 nt, synthetic construct
  source 1..20: mol_type = other RNA
ccctgtcctccaggctgtag

SEQ ID NO: 21657 - RNA, 20 nt, synthetic construct
  source 1..20: mol_type = other RNA
tgtcctccaggctgtagggg

SEQ ID NO: 21658 - RNA, 20 nt, synthetic construct
  source 1..20: mol_type = other RNA
cccctacagcctggaggaca

SEQ ID NO: 21659 - RNA, 20 nt, synthetic construct
  source 1..20: mol_type = other RNA
tcccctacagcctggaggac

SEQ ID NO: 21660 - RNA, 20 nt, synthetic construct
  source 1..20: mol_type = other RNA
tctcctcccctacagcctgg

SEQ ID NO: 21661 - RNA, 20 nt, synthetic construct
  source 1..20: mol_type = other RNA
ggctgtaggggaggagagcc

SEQ ID NO: 21662 - RNA, 20 nt, synthetic construct
  source 1..20: mol_type = other RNA
ggctctcctcccctacagcc

SEQ ID NO: 21663 - RNA, 20 nt, synthetic construct
  source 1..20: mol_type = other RNA
gtaggggaggagagcctggc

SEQ ID NO: 21664 - RNA, 20 nt, synthetic construct
  source 1..20: mol_type = other RNA
taggggaggagagcctggcc

SEQ ID NO: 21665 - RNA, 20 nt, synthetic construct
  source 1..20: mol_type = other RNA
aggggaggagagcctggccg

SEQ ID NO: 21666 - RNA, 20 nt, synthetic construct
  source 1..20: mol_type = other RNA
ggggaggagagcctggccgg

SEQ ID NO: 21667 - RNA, 20 nt, synthetic construct
  source 1..20: mol_type = other RNA
cctggccgggggagacagac

SEQ ID NO: 21668 - RNA, 20 nt, synthetic construct
  source 1..20: mol_type = other RNA
ccagtctgtctcccccggcc

SEQ ID NO: 21669 - RNA, 20 nt, synthetic construct
  source 1..20: mol_type = other RNA
aatgtccagtctgtctcccc

SEQ ID NO: 21670 - RNA, 20 nt, synthetic construct
  source 1..20: mol_type = other RNA
acatttccctgtttcgagcc

SEQ ID NO: 21671 - RNA, 20 nt, synthetic construct
  source 1..20: mol_type = other RNA
gaagagcctggctcgaaaca

SEQ ID NO: 21672 - RNA, 20 nt, synthetic construct
  source 1..20: mol_type = other RNA
ttcgagccaggctcttccaa

SEQ ID NO: 21673 - RNA, 20 nt, synthetic construct
  source 1..20: mol_type = other RNA
tcgagccaggctcttccaag

SEQ ID NO: 21674 - RNA, 20 nt, synthetic construct
  source 1..20: mol_type = other RNA
ggctcttccaaggggccagc

SEQ ID NO: 21675 - RNA, 20 nt, synthetic construct
  source 1..20: mol_type = other RNA
gctcttccaaggggccagct

SEQ ID NO: 21676 - RNA, 20 nt, synthetic construct
  source 1..20: mol_type = other RNA
gctggccccttggaagagcc

SEQ ID NO: 21677 - RNA, 20 nt, synthetic construct
  source 1..20: mol_type = other RNA
caaggggccagctgggtccc

SEQ ID NO: 21678 - RNA, 20 nt, synthetic construct
  source 1..20: mol_type = other RNA
cggggacccagctggcccct

SEQ ID NO: 21679 - RNA, 20 nt, synthetic construct
  source 1..20: mol_type = other RNA
actgactccggggacccagc

SEQ ID NO: 21680 - RNA, 20 nt, synthetic construct
  source 1..20: mol_type = other RNA
gggtccccggagtcagtcct

SEQ ID NO: 21681 - RNA, 20 nt, synthetic construct
  source 1..20: mol_type = other RNA
ccccggagtcagtcctaggc

SEQ ID NO: 21682 - RNA, 20 nt, synthetic construct
  source 1..20: mol_type = other RNA
ggagtcagtcctaggctgga

SEQ ID NO: 21683 - RNA, 20 nt, synthetic construct
  source 1..20: mol_type = other RNA
ccagcctaggactgactccg

SEQ ID NO: 21684 - RNA, 20 nt, synthetic construct
  source 1..20: mol_type = other RNA
tccagcctaggactgactcc

SEQ ID NO: 21685 - RNA, 20 nt, synthetic construct
  source 1..20: mol_type = other RNA
atccagcctaggactgactc

SEQ ID NO: 21686 - RNA, 20 nt, synthetic construct
  source 1..20: mol_type = other RNA
tcagtcctaggctggatggg

SEQ ID NO: 21687 - RNA, 20 nt, synthetic construct
  source 1..20: mol_type = other RNA
cagtcctaggctggatggga

SEQ ID NO: 21688 - RNA, 20 nt, synthetic construct
  source 1..20: mol_type = other RNA
tcctaggctggatgggaggg

SEQ ID NO: 21689 - RNA, 20 nt, synthetic construct
  source 1..20: mol_type = other RNA
gccaccctcccatccagcct

SEQ ID NO: 21690 - RNA, 20 nt, synthetic construct
  source 1..20: mol_type = other RNA
gggagggtggccccctcaag

SEQ ID NO: 21691 - RNA, 20 nt, synthetic construct
  source 1..20: mol_type = other RNA
ggctgggagtcctcttgagg

SEQ ID NO: 21692 - RNA, 20 nt, synthetic construct
  source 1..20: mol_type = other RNA
aggctgggagtcctcttgag

SEQ ID NO: 21693 - RNA, 20 nt, synthetic construct
  source 1..20: mol_type = other RNA
gaggctgggagtcctcttga

SEQ ID NO: 21694 - RNA, 20 nt, synthetic construct
  source 1..20: mol_type = other RNA
ggaggctgggagtcctcttg

SEQ ID NO: 21695 - RNA, 20 nt, synthetic construct
  source 1..20: mol_type = other RNA
ggactcccagcctccacatc

SEQ ID NO: 21696 - RNA, 20 nt, synthetic construct
  source 1..20: mol_type = other RNA
aggaaccagatgtggaggct

SEQ ID NO: 21697 - RNA, 20 nt, synthetic construct
  source 1..20: mol_type = other RNA
taggaaccagatgtggaggc

SEQ ID NO: 21698 - RNA, 20 nt, synthetic construct
  source 1..20: mol_type = other RNA
aaggtaggaaccagatgtgg

SEQ ID NO: 21699 - RNA, 20 nt, synthetic construct
  source 1..20: mol_type = other RNA
gtgaaggtaggaaccagatg

SEQ ID NO: 21700 - RNA, 20 nt, synthetic construct
  source 1..20: mol_type = other RNA
ggagggtgagatgtgaaggt

SEQ ID NO: 21701 - RNA, 20 nt, synthetic construct
  source 1..20: mol_type = other RNA
cacatctcaccctcccgttc

SEQ ID NO: 21702 - RNA, 20 nt, synthetic construct
  source 1..20: mol_type = other RNA
acatctcaccctcccgttct

SEQ ID NO: 21703 - RNA, 20 nt, synthetic construct
  source 1..20: mol_type = other RNA
catctcaccctcccgttctg

SEQ ID NO: 21704 - RNA, 20 nt, synthetic construct
  source 1..20: mol_type = other RNA
aattcttccccagaacggga

SEQ ID NO: 21705 - RNA, 20 nt, synthetic construct
  source 1..20: mol_type = other RNA
aaattcttccccagaacggg

SEQ ID NO: 21706 - RNA, 20 nt, synthetic construct
  source 1..20: mol_type = other RNA
cagaaattcttccccagaac

SEQ ID NO: 21707 - RNA, 20 nt, synthetic construct
  source 1..20: mol_type = other RNA
ccagaaattcttccccagaa

SEQ ID NO: 21708 - RNA, 20 nt, synthetic construct
  source 1..20: mol_type = other RNA
cagtatccactccatcctca

SEQ ID NO: 21709 - RNA, 20 nt, synthetic construct
  source 1..20: mol_type = other RNA
gaggatggagtggatactgt

SEQ ID NO: 21710 - RNA, 20 nt, synthetic construct
  source 1..20: mol_type = other RNA
ccatcctcaaggcttcccgc

SEQ ID NO: 21711 - RNA, 20 nt, synthetic construct
  source 1..20: mol_type = other RNA
catcctcaaggcttcccgca

SEQ ID NO: 21712 - RNA, 20 nt, synthetic construct
  source 1..20: mol_type = other RNA
cctgcgggaagccttgagga

SEQ ID NO: 21713 - RNA, 20 nt, synthetic construct
  source 1..20: mol_type = other RNA
caaggcttcccgcagggcct

SEQ ID NO: 21714 - RNA, 20 nt, synthetic construct
  source 1..20: mol_type = other RNA
aaggcttcccgcagggcctt

SEQ ID NO: 21715 - RNA, 20 nt, synthetic construct
  source 1..20: mol_type = other RNA
aggcttcccgcagggccttg

SEQ ID NO: 21716 - RNA, 20 nt, synthetic construct
  source 1..20: mol_type = other RNA
gcagtgccccaaggccctgc

SEQ ID NO: 21717 - RNA, 20 nt, synthetic construct
  source 1..20: mol_type = other RNA
ggcagtgccccaaggccctg

SEQ ID NO: 21718 - RNA, 20 nt, synthetic construct
  source 1..20: mol_type = other RNA
ttggggcactgccttgccat

SEQ ID NO: 21719 - RNA, 20 nt, synthetic construct
  source 1..20: mol_type = other RNA
tggggcactgccttgccatc

SEQ ID NO: 21720 - RNA, 20 nt, synthetic construct
  source 1..20: mol_type = other RNA
gatggcaaggcagtgcccca

SEQ ID NO: 21721 - RNA, 20 nt, synthetic construct
  source 1..20: mol_type = other RNA
tgccatcgggcccagttctc

SEQ ID NO: 21722 - RNA, 20 nt, synthetic construct
  source 1..20: mol_type = other RNA
gccatcgggcccagttctcc

SEQ ID NO: 21723 - RNA, 20 nt, synthetic construct
  source 1..20: mol_type = other RNA
gagaactgggcccgatggca

SEQ ID NO: 21724 - RNA, 20 nt, synthetic construct
  source 1..20: mol_type = other RNA
gcccggagaactgggcccga

SEQ ID NO: 21725 - RNA, 20 nt, synthetic construct
  source 1..20: mol_type = other RNA
caggtggggcccggagaact

SEQ ID NO: 21726 - RNA, 20 nt, synthetic construct
  source 1..20: mol_type = other RNA
gcaggtggggcccggagaac

SEQ ID NO: 21727 - RNA, 20 nt, synthetic construct
  source 1..20: mol_type = other RNA
aaaggggtgcaggtggggcc

SEQ ID NO: 21728 - RNA, 20 nt, synthetic construct
  source 1..20: mol_type = other RNA
ggaagaaaggggtgcaggtg

SEQ ID NO: 21729 - RNA, 20 nt, synthetic construct
  source 1..20: mol_type = other RNA
gggaagaaaggggtgcaggt

SEQ ID NO: 21730 - RNA, 20 nt, synthetic construct
  source 1..20: mol_type = other RNA
tgcacccctttcttccccct

SEQ ID NO: 21731 - RNA, 20 nt, synthetic construct
  source 1..20: mol_type = other RNA
cagggggaagaaaggggtgc

SEQ ID NO: 21732 - RNA, 20 nt, synthetic construct
  source 1..20: mol_type = other RNA
atatcccagggggaagaaag

SEQ ID NO: 21733 - RNA, 20 nt, synthetic construct
  source 1..20: mol_type = other RNA
catatcccagggggaagaaa

SEQ ID NO: 21734 - RNA, 20 nt, synthetic construct
  source 1..20: mol_type = other RNA
tcatatcccagggggaagaa

SEQ ID NO: 21735 - RNA, 20 nt, synthetic construct
  source 1..20: mol_type = other RNA
tccccctgggatatgatgtg

SEQ ID NO: 21736 - RNA, 20 nt, synthetic construct
  source 1..20: mol_type = other RNA
accacacatcatatcccagg

SEQ ID NO: 21737 - RNA, 20 nt, synthetic construct
  source 1..20: mol_type = other RNA
caccacacatcatatcccag

SEQ ID NO: 21738 - RNA, 20 nt, synthetic construct
  source 1..20: mol_type = other RNA
acaccacacatcatatccca

SEQ ID NO: 21739 - RNA, 20 nt, synthetic construct
  source 1..20: mol_type = other RNA
aacaccacacatcatatccc

SEQ ID NO: 21740 - RNA, 20 nt, synthetic construct
  source 1..20: mol_type = other RNA
atgatgtgtggtgtttcctg

SEQ ID NO: 21741 - RNA, 20 nt, synthetic construct
  source 1..20: mol_type = other RNA
tttcctgtggtaaaagactg

SEQ ID NO: 21742 - RNA, 20 nt, synthetic construct
  source 1..20: mol_type = other RNA
ctgtggtaaaagactgaggc

SEQ ID NO: 21743 - RNA, 20 nt, synthetic construct
  source 1..20: mol_type = other RNA
ctgcctcagtcttttaccac

SEQ ID NO: 21744 - RNA, 20 nt, synthetic construct
  source 1..20: mol_type = other RNA
gtaaaagactgaggcaggcc

SEQ ID NO: 21745 - RNA, 20 nt, synthetic construct
  source 1..20: mol_type = other RNA
taaaagactgaggcaggcca

SEQ ID NO: 21746 - RNA, 20 nt, synthetic construct
  source 1..20: mol_type = other RNA
aaaagactgaggcaggccag

SEQ ID NO: 21747 - RNA, 20 nt, synthetic construct
  source 1..20: mol_type = other RNA
acatgttactggcagacccc

SEQ ID NO: 21748 - RNA, 20 nt, synthetic construct
  source 1..20: mol_type = other RNA
tgtacatgggaacatgttac

SEQ ID NO: 21749 - RNA, 20 nt, synthetic construct
  source 1..20: mol_type = other RNA
catgttcccatgtacagaca

SEQ ID NO: 21750 - RNA, 20 nt, synthetic construct
  source 1..20: mol_type = other RNA
tggggaccgtgtctgtacat

SEQ ID NO: 21751 - RNA, 20 nt, synthetic construct
  source 1..20: mol_type = other RNA
gtggggaccgtgtctgtaca

SEQ ID NO: 21752 - RNA, 20 nt, synthetic construct
  source 1..20: mol_type = other RNA
ccccacaccctcccagcctc

SEQ ID NO: 21753 - RNA, 20 nt, synthetic construct
  source 1..20: mol_type = other RNA
cctgaggctgggagggtgtg

SEQ ID NO: 21754 - RNA, 20 nt, synthetic construct
  source 1..20: mol_type = other RNA
accctcccagcctcaggccc

SEQ ID NO: 21755 - RNA, 20 nt, synthetic construct
  source 1..20: mol_type = other RNA
ggcctgaggctgggagggtg

SEQ ID NO: 21756 - RNA, 20 nt, synthetic construct
  source 1..20: mol_type = other RNA
gcctgggcctgaggctggga

SEQ ID NO: 21757 - RNA, 20 nt, synthetic construct
  source 1..20: mol_type = other RNA
tgcctgggcctgaggctggg

SEQ ID NO: 21758 - RNA, 20 nt, synthetic construct
  source 1..20: mol_type = other RNA
gcctcaggcccaggcagaca

SEQ ID NO: 21759 - RNA, 20 nt, synthetic construct
  source 1..20: mol_type = other RNA
gtctgcctgggcctgaggct

SEQ ID NO: 21760 - RNA, 20 nt, synthetic construct
  source 1..20: mol_type = other RNA
tgtctgcctgggcctgaggc

SEQ ID NO: 21761 - RNA, 20 nt, synthetic construct
  source 1..20: mol_type = other RNA
cccatgtctgcctgggcctg

SEQ ID NO: 21762 - RNA, 20 nt, synthetic construct
  source 1..20: mol_type = other RNA
ccaggcagacatgggcgagc

SEQ ID NO: 21763 - RNA, 20 nt, synthetic construct
  source 1..20: mol_type = other RNA
cagctcgcccatgtctgcct

SEQ ID NO: 21764 - RNA, 20 nt, synthetic construct
  source 1..20: mol_type = other RNA
ccagctcgcccatgtctgcc

SEQ ID NO: 21765 - RNA, 20 nt, synthetic construct
  source 1..20: mol_type = other RNA
gctggtgagactgccagcca

SEQ ID NO: 21766 - RNA, 20 nt, synthetic construct
  source 1..20: mol_type = other RNA
tggctaagcaaagccgtggc

SEQ ID NO: 21767 - RNA, 20 nt, synthetic construct
  source 1..20: mol_type = other RNA
cggctttgcttagccacctg

SEQ ID NO: 21768 - RNA, 20 nt, synthetic construct
  source 1..20: mol_type = other RNA
caggtggctaagcaaagccg

SEQ ID NO: 21769 - RNA, 20 nt, synthetic construct
  source 1..20: mol_type = other RNA
tgcttagccacctgtggccg

SEQ ID NO: 21770 - RNA, 20 nt, synthetic construct
  source 1..20: mol_type = other RNA
gcttagccacctgtggccga

SEQ ID NO: 21771 - RNA, 20 nt, synthetic construct
  source 1..20: mol_type = other RNA
tgagagccctcggccacagg

SEQ ID NO: 21772 - RNA, 20 nt, synthetic construct
  source 1..20: mol_type = other RNA
ctctgagagccctcggccac

SEQ ID NO: 21773 - RNA, 20 nt, synthetic construct
  source 1..20: mol_type = other RNA
agggggtctctgagagccct

SEQ ID NO: 21774 - RNA, 20 nt, synthetic construct
  source 1..20: mol_type = other RNA
tagtatttgggaggttaagg

SEQ ID NO: 21775 - RNA, 20 nt, synthetic construct
  source 1..20: mol_type = other RNA
ttagtatttgggaggttaag

SEQ ID NO: 21776 - RNA, 20 nt, synthetic construct
  source 1..20: mol_type = other RNA
cttagtatttgggaggttaa

SEQ ID NO: 21777 - RNA, 20 nt, synthetic construct
  source 1..20: mol_type = other RNA
tcttagtatttgggaggtta

SEQ ID NO: 21778 - RNA, 20 nt, synthetic construct
  source 1..20: mol_type = other RNA
ttagcttcttagtatttggg

SEQ ID NO: 21779 - RNA, 20 nt, synthetic construct
  source 1..20: mol_type = other RNA
attttagcttcttagtattt

SEQ ID NO: 21780 - RNA, 20 nt, synthetic construct
  source 1..20: mol_type = other RNA
tattttagcttcttagtatt

SEQ ID NO: 21781 - RNA, 20 nt, synthetic construct
  source 1..20: mol_type = other RNA
tattttgtttttttttttct

SEQ ID NO: 21782 - RNA, 20 nt, synthetic construct
  source 1..20: mol_type = other RNA
tggtgccagagtttataccc

SEQ ID NO: 21783 - RNA, 20 nt, synthetic construct
  source 1..20: mol_type = other RNA
ggtgccagagtttataccct

SEQ ID NO: 21784 - RNA, 20 nt, synthetic construct
  source 1..20: mol_type = other RNA
agagtttataccctgggtgc

SEQ ID NO: 21785 - RNA, 20 nt, synthetic construct
  source 1..20: mol_type = other RNA
gagtttataccctgggtgct

SEQ ID NO: 21786 - RNA, 20 nt, synthetic construct
  source 1..20: mol_type = other RNA
agtttataccctgggtgctg

SEQ ID NO: 21787 - RNA, 20 nt, synthetic construct
  source 1..20: mol_type = other RNA
agcacccagggtataaactc

SEQ ID NO: 21788 - RNA, 20 nt, synthetic construct
  source 1..20: mol_type = other RNA
cagtgcgaccccagcaccca

SEQ ID NO: 21789 - RNA, 20 nt, synthetic construct
  source 1..20: mol_type = other RNA
acagtgcgaccccagcaccc

SEQ ID NO: 21790 - RNA, 20 nt, synthetic construct
  source 1..20: mol_type = other RNA
tatatatattctattttttt

SEQ ID NO: 21791 - RNA, 20 nt, synthetic construct
  source 1..20: mol_type = other RNA
tatattctattttttttggt

SEQ ID NO: 21792 - RNA, 20 nt, synthetic construct
  source 1..20: mol_type = other RNA
atattctattttttttggtt

SEQ ID NO: 21793 - RNA, 20 nt, synthetic construct
  source 1..20: mol_type = other RNA
tttaattcagtcctacaaaa

SEQ ID NO: 21794 - RNA, 20 nt, synthetic construct
  source 1..20: mol_type = other RNA
aattcagtcctacaaaatgg

SEQ ID NO: 21795 - RNA, 20 nt, synthetic construct
  source 1..20: mol_type = other RNA
ggggcttaccaccattttgt

SEQ ID NO: 21796 - RNA, 20 nt, synthetic construct
  source 1..20: mol_type = other RNA
tggtggtaagccccagtctc

SEQ ID NO: 21797 - RNA, 20 nt, synthetic construct
  source 1..20: mol_type = other RNA
ggtggtaagccccagtctca

SEQ ID NO: 21798 - RNA, 20 nt, synthetic construct
  source 1..20: mol_type = other RNA
gtggtaagccccagtctcag

SEQ ID NO: 21799 - RNA, 20 nt, synthetic construct
  source 1..20: mol_type = other RNA
cagggtgacccctgagactg

SEQ ID NO: 21800 - RNA, 20 nt, synthetic construct
  source 1..20: mol_type = other RNA
acagggtgacccctgagact

SEQ ID NO: 21801 - RNA, 20 nt, synthetic construct
  source 1..20: mol_type = other RNA
gacagggtgacccctgagac

SEQ ID NO: 21802 - RNA, 20 nt, synthetic construct
  source 1..20: mol_type = other RNA
ctgtcttagagctagagatg

SEQ ID NO: 21803 - RNA, 20 nt, synthetic construct
  source 1..20: mol_type = other RNA
tcttagagctagagatgagg

SEQ ID NO: 21804 - RNA, 20 nt, synthetic construct
  source 1..20: mol_type = other RNA
ctcatctctagctctaagac

SEQ ID NO: 21805 - RNA, 20 nt, synthetic construct
  source 1..20: mol_type = other RNA
agagctagagatgaggtggc

SEQ ID NO: 21806 - RNA, 20 nt, synthetic construct
  source 1..20: mol_type = other RNA
gagctagagatgaggtggca

SEQ ID NO: 21807 - RNA, 20 nt, synthetic construct
  source 1..20: mol_type = other RNA
ctagagatgaggtggcaggg

SEQ ID NO: 21808 - RNA, 20 nt, synthetic construct
  source 1..20: mol_type = other RNA
tagagatgaggtggcaggga

SEQ ID NO: 21809 - RNA, 20 nt, synthetic construct
  source 1..20: mol_type = other RNA
agatgaggtggcagggaggg

SEQ ID NO: 21810 - RNA, 20 nt, synthetic construct
  source 1..20: mol_type = other RNA
gagggaggctgtgtcctcag

SEQ ID NO: 21811 - RNA, 20 nt, synthetic construct
  source 1..20: mol_type = other RNA
aggctgtgtcctcagtggcc

SEQ ID NO: 21812 - RNA, 20 nt, synthetic construct
  source 1..20: mol_type = other RNA
ggctgtgtcctcagtggcct

SEQ ID NO: 21813 - RNA, 20 nt, synthetic construct
  source 1..20: mol_type = other RNA
gctgtgtcctcagtggcctg

SEQ ID NO: 21814 - RNA, 20 nt, synthetic construct
  source 1..20: mol_type = other RNA
tgctcagccccaggccactg

SEQ ID NO: 21815 - RNA, 20 nt, synthetic construct
  source 1..20: mol_type = other RNA
cctggggctgagcagacctt

SEQ ID NO: 21816 - RNA, 20 nt, synthetic construct
  source 1..20: mol_type = other RNA
gggctgagcagaccttagga

SEQ ID NO: 21817 - RNA, 20 nt, synthetic construct
  source 1..20: mol_type = other RNA
ggctgagcagaccttaggaa

SEQ ID NO: 21818 - RNA, 20 nt, synthetic construct
  source 1..20: mol_type = other RNA
gctgagcagaccttaggaag

SEQ ID NO: 21819 - RNA, 20 nt, synthetic construct
  source 1..20: mol_type = other RNA
ctggggagggccccttccta

SEQ ID NO: 21820 - RNA, 20 nt, synthetic construct
  source 1..20: mol_type = other RNA
aggggccctccccagtgccg

SEQ ID NO: 21821 - RNA, 20 nt, synthetic construct
  source 1..20: mol_type = other RNA
ccccagtgccgtggctgctc

SEQ ID NO: 21822 - RNA, 20 nt, synthetic construct
  source 1..20: mol_type = other RNA
agcagccacggcactgggga

SEQ ID NO: 21823 - RNA, 20 nt, synthetic construct
  source 1..20: mol_type = other RNA
gagcagccacggcactgggg

SEQ ID NO: 21824 - RNA, 20 nt, synthetic construct
  source 1..20: mol_type = other RNA
ccagagcagccacggcactg

SEQ ID NO: 21825 - RNA, 20 nt, synthetic construct
  source 1..20: mol_type = other RNA
cccagagcagccacggcact

SEQ ID NO: 21826 - RNA, 20 nt, synthetic construct
  source 1..20: mol_type = other RNA
ccccagagcagccacggcac

SEQ ID NO: 21827 - RNA, 20 nt, synthetic construct
  source 1..20: mol_type = other RNA
ggctgctctggggctacccc

SEQ ID NO: 21828 - RNA, 20 nt, synthetic construct
  source 1..20: mol_type = other RNA
gggtagccccagagcagcca

SEQ ID NO: 21829 - RNA, 20 nt, synthetic construct
  source 1..20: mol_type = other RNA
gggctaccccaggtgaacag

SEQ ID NO: 21830 - RNA, 20 nt, synthetic construct
  source 1..20: mol_type = other RNA
ctaccccaggtgaacagagg

SEQ ID NO: 21831 - RNA, 20 nt, synthetic construct
  source 1..20: mol_type = other RNA
tcaccacctctgttcacctg

SEQ ID NO: 21832 - RNA, 20 nt, synthetic construct
  source 1..20: mol_type = other RNA
ctcaccacctctgttcacct

SEQ ID NO: 21833 - RNA, 20 nt, synthetic construct
  source 1..20: mol_type = other RNA
tctcaccacctctgttcacc

SEQ ID NO: 21834 - RNA, 20 nt, synthetic construct
  source 1..20: mol_type = other RNA
acagaggtggtgagatgcgc

SEQ ID NO: 21835 - RNA, 20 nt, synthetic construct
  source 1..20: mol_type = other RNA
cagaggtggtgagatgcgca

SEQ ID NO: 21836 - RNA, 20 nt, synthetic construct
  source 1..20: mol_type = other RNA
agggaagaccagctctctcc

SEQ ID NO: 21837 - RNA, 20 nt, synthetic construct
  source 1..20: mol_type = other RNA
accagctctctccaggacat

SEQ ID NO: 21838 - RNA, 20 nt, synthetic construct
  source 1..20: mol_type = other RNA
ccagctctctccaggacatc

SEQ ID NO: 21839 - RNA, 20 nt, synthetic construct
  source 1..20: mol_type = other RNA
cccgatgtcctggagagagc

SEQ ID NO: 21840 - RNA, 20 nt, synthetic construct
  source 1..20: mol_type = other RNA
cttcacgcagcccgatgtcc

SEQ ID NO: 21841 - RNA, 20 nt, synthetic construct
  source 1..20: mol_type = other RNA
cgtgaagtccagtgaccctg

SEQ ID NO: 21842 - RNA, 20 nt, synthetic construct
  source 1..20: mol_type = other RNA
gtgaagtccagtgaccctga

SEQ ID NO: 21843 - RNA, 20 nt, synthetic construct
  source 1..20: mol_type = other RNA
tgaagtccagtgaccctgag

SEQ ID NO: 21844 - RNA, 20 nt, synthetic construct
  source 1..20: mol_type = other RNA
cagtgaccctgaggggattt

SEQ ID NO: 21845 - RNA, 20 nt, synthetic construct
  source 1..20: mol_type = other RNA
caaaatcccctcagggtcac

SEQ ID NO: 21846 - RNA, 20 nt, synthetic construct
  source 1..20: mol_type = other RNA
cctgaggggattttggccaa

SEQ ID NO: 21847 - RNA, 20 nt, synthetic construct
  source 1..20: mol_type = other RNA
ctttggccaaaatcccctca

SEQ ID NO: 21848 - RNA, 20 nt, synthetic construct
  source 1..20: mol_type = other RNA
cctttggccaaaatcccctc

SEQ ID NO: 21849 - RNA, 20 nt, synthetic construct
  source 1..20: mol_type = other RNA
tttggccaaaggaaacagcc

SEQ ID NO: 21850 - RNA, 20 nt, synthetic construct
  source 1..20: mol_type = other RNA
ttggccaaaggaaacagcca

SEQ ID NO: 21851 - RNA, 20 nt, synthetic construct
  source 1..20: mol_type = other RNA
ccaaaggaaacagccagggc

SEQ ID NO: 21852 - RNA, 20 nt, synthetic construct
  source 1..20: mol_type = other RNA
caaaggaaacagccagggct

SEQ ID NO: 21853 - RNA, 20 nt, synthetic construct
  source 1..20: mol_type = other RNA
ccagccctggctgtttcctt

SEQ ID NO: 21854 - RNA, 20 nt, synthetic construct
  source 1..20: mol_type = other RNA
gaaacagccagggctgggct

SEQ ID NO: 21855 - RNA, 20 nt, synthetic construct
  source 1..20: mol_type = other RNA
cagggctgggctaggagagc

SEQ ID NO: 21856 - RNA, 20 nt, synthetic construct
  source 1..20: mol_type = other RNA
agggctgggctaggagagct

SEQ ID NO: 21857 - RNA, 20 nt, synthetic construct
  source 1..20: mol_type = other RNA
gggctgggctaggagagctg

SEQ ID NO: 21858 - RNA, 20 nt, synthetic construct
  source 1..20: mol_type = other RNA
cagctctcctagcccagccc

SEQ ID NO: 21859 - RNA, 20 nt, synthetic construct
  source 1..20: mol_type = other RNA
cccacccactctccctcaca

SEQ ID NO: 21860 - RNA, 20 nt, synthetic construct
  source 1..20: mol_type = other RNA
catgtgagggagagtgggtg

SEQ ID NO: 21861 - RNA, 20 nt, synthetic construct
  source 1..20: mol_type = other RNA
ccatgtgagggagagtgggt

SEQ ID NO: 21862 - RNA, 20 nt, synthetic construct
  source 1..20: mol_type = other RNA
accatgtgagggagagtggg

SEQ ID NO: 21863 - RNA, 20 nt, synthetic construct
  source 1..20: mol_type = other RNA
actctccctcacatggtgct

SEQ ID NO: 21864 - RNA, 20 nt, synthetic construct
  source 1..20: mol_type = other RNA
agcaccatgtgagggagagt

SEQ ID NO: 21865 - RNA, 20 nt, synthetic construct
  source 1..20: mol_type = other RNA
tagcaccatgtgagggagag

SEQ ID NO: 21866 - RNA, 20 nt, synthetic construct
  source 1..20: mol_type = other RNA
tccctcacatggtgctaggc

SEQ ID NO: 21867 - RNA, 20 nt, synthetic construct
  source 1..20: mol_type = other RNA
ccctcacatggtgctaggct

SEQ ID NO: 21868 - RNA, 20 nt, synthetic construct
  source 1..20: mol_type = other RNA
cccagcctagcaccatgtga

SEQ ID NO: 21869 - RNA, 20 nt, synthetic construct
  source 1..20: mol_type = other RNA
tcccagcctagcaccatgtg

SEQ ID NO: 21870 - RNA, 20 nt, synthetic construct
  source 1..20: mol_type = other RNA
ctgggagctgccctgagagc

SEQ ID NO: 21871 - RNA, 20 nt, synthetic construct
  source 1..20: mol_type = other RNA
tgggagctgccctgagagct

SEQ ID NO: 21872 - RNA, 20 nt, synthetic construct
  source 1..20: mol_type = other RNA
gagagctgggatgcccacca

SEQ ID NO: 21873 - RNA, 20 nt, synthetic construct
  source 1..20: mol_type = other RNA
ggtgggcatcccagctctca

SEQ ID NO: 21874 - RNA, 20 nt, synthetic construct
  source 1..20: mol_type = other RNA
tggtgggcatcccagctctc

SEQ ID NO: 21875 - RNA, 20 nt, synthetic construct
  source 1..20: mol_type = other RNA
acagttctgtgggccttggt

SEQ ID NO: 21876 - RNA, 20 nt, synthetic construct
  source 1..20: mol_type = other RNA
gacagttctgtgggccttgg

SEQ ID NO: 21877 - RNA, 20 nt, synthetic construct
  source 1..20: mol_type = other RNA
aggcccacagaactgtctcc

SEQ ID NO: 21878 - RNA, 20 nt, synthetic construct
  source 1..20: mol_type = other RNA
ggagacagttctgtgggcct

SEQ ID NO: 21879 - RNA, 20 nt, synthetic construct
  source 1..20: mol_type = other RNA
gggcctggagacagttctgt

SEQ ID NO: 21880 - RNA, 20 nt, synthetic construct
  source 1..20: mol_type = other RNA
agggcctggagacagttctg

SEQ ID NO: 21881 - RNA, 20 nt, synthetic construct
  source 1..20: mol_type = other RNA
ctccaggcccttgtagacag

SEQ ID NO: 21882 - RNA, 20 nt, synthetic construct
  source 1..20: mol_type = other RNA
tccaggcccttgtagacagt

SEQ ID NO: 21883 - RNA, 20 nt, synthetic construct
  source 1..20: mol_type = other RNA
tcccactgtctacaagggcc

SEQ ID NO: 21884 - RNA, 20 nt, synthetic construct
  source 1..20: mol_type = other RNA
cttgtagacagtgggatctc

SEQ ID NO: 21885 - RNA, 20 nt, synthetic construct
  source 1..20: mol_type = other RNA
ttgtagacagtgggatctct

SEQ ID NO: 21886 - RNA, 20 nt, synthetic construct
  source 1..20: mol_type = other RNA
agagatcccactgtctacaa

SEQ ID NO: 21887 - RNA, 20 nt, synthetic construct
  source 1..20: mol_type = other RNA
cagagatcccactgtctaca

SEQ ID NO: 21888 - RNA, 20 nt, synthetic construct
  source 1..20: mol_type = other RNA
gggatctctgggctgatttc

SEQ ID NO: 21889 - RNA, 20 nt, synthetic construct
  source 1..20: mol_type = other RNA
tctctgggctgatttctggt

SEQ ID NO: 21890 - RNA, 20 nt, synthetic construct
  source 1..20: mol_type = other RNA
ctctgggctgatttctggtt

SEQ ID NO: 21891 - RNA, 20 nt, synthetic construct
  source 1..20: mol_type = other RNA
tctgggctgatttctggttg

SEQ ID NO: 21892 - RNA, 20 nt, synthetic construct
  source 1..20: mol_type = other RNA
attgttaaatggggtggggt

SEQ ID NO: 21893 - RNA, 20 nt, synthetic construct
  source 1..20: mol_type = other RNA
tcacattgttaaatggggtg

SEQ ID NO: 21894 - RNA, 20 nt, synthetic construct
  source 1..20: mol_type = other RNA
ttcacattgttaaatggggt

SEQ ID NO: 21895 - RNA, 20 nt, synthetic construct
  source 1..20: mol_type = other RNA
cttcacattgttaaatgggg

SEQ ID NO: 21896 - RNA, 20 nt, synthetic construct
  source 1..20: mol_type = other RNA
tcacttcacattgttaaatg

SEQ ID NO: 21897 - RNA, 20 nt, synthetic construct
  source 1..20: mol_type = other RNA
gtcacttcacattgttaaat

SEQ ID NO: 21898 - RNA, 20 nt, synthetic construct
  source 1..20: mol_type = other RNA
agtcacttcacattgttaaa

SEQ ID NO: 21899 - RNA, 20 nt, synthetic construct
  source 1..20: mol_type = other RNA
caatgtgaagtgactgaggc

SEQ ID NO: 21900 - RNA, 20 nt, synthetic construct
  source 1..20: mol_type = other RNA
aatgtgaagtgactgaggct

SEQ ID NO: 21901 - RNA, 20 nt, synthetic construct
  source 1..20: mol_type = other RNA
atgtgaagtgactgaggctg

SEQ ID NO: 21902 - RNA, 20 nt, synthetic construct
  source 1..20: mol_type = other RNA
gaggctggggtgcctctccc

SEQ ID NO: 21903 - RNA, 20 nt, synthetic construct
  source 1..20: mol_type = other RNA
agttggagggggccagggag

SEQ ID NO: 21904 - RNA, 20 nt, synthetic construct
  source 1..20: mol_type = other RNA
ttggcagttggagggggcca

SEQ ID NO: 21905 - RNA, 20 nt, synthetic construct
  source 1..20: mol_type = other RNA
tttggcagttggagggggcc

SEQ ID NO: 21906 - RNA, 20 nt, synthetic construct
  source 1..20: mol_type = other RNA
cagaatttggcagttggagg

SEQ ID NO: 21907 - RNA, 20 nt, synthetic construct
  source 1..20: mol_type = other RNA
gcagaatttggcagttggag

SEQ ID NO: 21908 - RNA, 20 nt, synthetic construct
  source 1..20: mol_type = other RNA
agcagaatttggcagttgga

SEQ ID NO: 21909 - RNA, 20 nt, synthetic construct
  source 1..20: mol_type = other RNA
aagcagaatttggcagttgg

SEQ ID NO: 21910 - RNA, 20 nt, synthetic construct
  source 1..20: mol_type = other RNA
gggaagcagaatttggcagt

SEQ ID NO: 21911 - RNA, 20 nt, synthetic construct
  source 1..20: mol_type = other RNA
gttcagagggaagcagaatt

SEQ ID NO: 21912 - RNA, 20 nt, synthetic construct
  source 1..20: mol_type = other RNA
tctgcttccctctgaacccc

SEQ ID NO: 21913 - RNA, 20 nt, synthetic construct
  source 1..20: mol_type = other RNA
agtatttcctggggttcaga

SEQ ID NO: 21914 - RNA, 20 nt, synthetic construct
  source 1..20: mol_type = other RNA
gaaccccaggaaatactttc

SEQ ID NO: 21915 - RNA, 20 nt, synthetic construct
  source 1..20: mol_type = other RNA
ccaggaaatactttctggag

SEQ ID NO: 21916 - RNA, 20 nt, synthetic construct
  source 1..20: mol_type = other RNA
tctccagaaagtatttcctg

SEQ ID NO: 21917 - RNA, 20 nt, synthetic construct
  source 1..20: mol_type = other RNA
ctctccagaaagtatttcct

SEQ ID NO: 21918 - RNA, 20 nt, synthetic construct
  source 1..20: mol_type = other RNA
cctctccagaaagtatttcc

SEQ ID NO: 21919 - RNA, 20 nt, synthetic construct
  source 1..20: mol_type = other RNA
ttcagaagactctagcatct

SEQ ID NO: 21920 - RNA, 20 nt, synthetic construct
  source 1..20: mol_type = other RNA
tcagaagactctagcatctt

SEQ ID NO: 21921 - RNA, 20 nt, synthetic construct
  source 1..20: mol_type = other RNA
cagaagactctagcatcttg

SEQ ID NO: 21922 - RNA, 20 nt, synthetic construct
  source 1..20: mol_type = other RNA
agactctagcatcttggggc

SEQ ID NO: 21923 - RNA, 20 nt, synthetic construct
  source 1..20: mol_type = other RNA
tctagcatcttggggctgga

SEQ ID NO: 21924 - RNA, 20 nt, synthetic construct
  source 1..20: mol_type = other RNA
ggggctggaaggtcctttga

SEQ ID NO: 21925 - RNA, 20 nt, synthetic construct
  source 1..20: mol_type = other RNA
gggctggaaggtcctttgac

SEQ ID NO: 21926 - RNA, 20 nt, synthetic construct
  source 1..20: mol_type = other RNA
tcctttgacgggtatgaaac

SEQ ID NO: 21927 - RNA, 20 nt, synthetic construct
  source 1..20: mol_type = other RNA
acctgtttcatacccgtcaa

SEQ ID NO: 21928 - RNA, 20 nt, synthetic construct
  source 1..20: mol_type = other RNA
ggtatgaaacaggtccagaa

SEQ ID NO: 21929 - RNA, 20 nt, synthetic construct
  source 1..20: mol_type = other RNA
gtatgaaacaggtccagaaa

SEQ ID NO: 21930 - RNA, 20 nt, synthetic construct
  source 1..20: mol_type = other RNA
tatgaaacaggtccagaaag

SEQ ID NO: 21931 - RNA, 20 nt, synthetic construct
  source 1..20: mol_type = other RNA
gaaacaggtccagaaagggg

SEQ ID NO: 21932 - RNA, 20 nt, synthetic construct
  source 1..20: mol_type = other RNA
acaggtccagaaaggggagg

SEQ ID NO: 21933 - RNA, 20 nt, synthetic construct
  source 1..20: mol_type = other RNA
gaaaggggaggtggcctgct

SEQ ID NO: 21934 - RNA, 20 nt, synthetic construct
  source 1..20: mol_type = other RNA
agcaggccacctcccctttc

SEQ ID NO: 21935 - RNA, 20 nt, synthetic construct
  source 1..20: mol_type = other RNA
ggcctgcttggccgacgtca

SEQ ID NO: 21936 - RNA, 20 nt, synthetic construct
  source 1..20: mol_type = other RNA
ctccatgacgtcggccaagc

SEQ ID NO: 21937 - RNA, 20 nt, synthetic construct
  source 1..20: mol_type = other RNA
gccgacgtcatggagccagc

SEQ ID NO: 21938 - RNA, 20 nt, synthetic construct
  source 1..20: mol_type = other RNA
ccgacgtcatggagccagct

SEQ ID NO: 21939 - RNA, 20 nt, synthetic construct
  source 1..20: mol_type = other RNA
cccagctggctccatgacgt

SEQ ID NO: 21940 - RNA, 20 nt, synthetic construct
  source 1..20: mol_type = other RNA
tcatggagccagctgggagc

SEQ ID NO: 21941 - RNA, 20 nt, synthetic construct
  source 1..20: mol_type = other RNA
catggagccagctgggagca

SEQ ID NO: 21942 - RNA, 20 nt, synthetic construct
  source 1..20: mol_type = other RNA
cgctcagccctgctcccagc

SEQ ID NO: 21943 - RNA, 20 nt, synthetic construct
  source 1..20: mol_type = other RNA
agggctgagcgttgaacccg

SEQ ID NO: 21944 - RNA, 20 nt, synthetic construct
  source 1..20: mol_type = other RNA
agcgttgaacccgaggctcc

SEQ ID NO: 21945 - RNA, 20 nt, synthetic construct
  source 1..20: mol_type = other RNA
gacttggaaccgggagcctc

SEQ ID NO: 21946 - RNA, 20 nt, synthetic construct
  source 1..20: mol_type = other RNA
ggacttggaaccgggagcct

SEQ ID NO: 21947 - RNA, 20 nt, synthetic construct
  source 1..20: mol_type = other RNA
gcacgatgggacttggaacc

SEQ ID NO: 21948 - RNA, 20 nt, synthetic construct
  source 1..20: mol_type = other RNA
agcacgatgggacttggaac

SEQ ID NO: 21949 - RNA, 20 nt, synthetic construct
  source 1..20: mol_type = other RNA
aagaggagcacgatgggact

SEQ ID NO: 21950 - RNA, 20 nt, synthetic construct
  source 1..20: mol_type = other RNA
cattggaagaggagcacgat

SEQ ID NO: 21951 - RNA, 20 nt, synthetic construct
  source 1..20: mol_type = other RNA
gcattggaagaggagcacga

SEQ ID NO: 21952 - RNA, 20 nt, synthetic construct
  source 1..20: mol_type = other RNA
aggcagtgtggcattggaag

SEQ ID NO: 21953 - RNA, 20 nt, synthetic construct
  source 1..20: mol_type = other RNA
gctcagaggcagtgtggcat

SEQ ID NO: 21954 - RNA, 20 nt, synthetic construct
  source 1..20: mol_type = other RNA
actgcctctgagcccatcct

SEQ ID NO: 21955 - RNA, 20 nt, synthetic construct
  source 1..20: mol_type = other RNA
ggatgggctcagaggcagtg

SEQ ID NO: 21956 - RNA, 20 nt, synthetic construct
  source 1..20: mol_type = other RNA
ggtcccaaggatgggctcag

SEQ ID NO: 21957 - RNA, 20 nt, synthetic construct
  source 1..20: mol_type = other RNA
cagagtagggtcccaaggat

SEQ ID NO: 21958 - RNA, 20 nt, synthetic construct
  source 1..20: mol_type = other RNA
acagagtagggtcccaagga

SEQ ID NO: 21959 - RNA, 20 nt, synthetic construct
  source 1..20: mol_type = other RNA
ttgggaccctactctgtgcc

SEQ ID NO: 21960 - RNA, 20 nt, synthetic construct
  source 1..20: mol_type = other RNA
tggcacagagtagggtccca

SEQ ID NO: 21961 - RNA, 20 nt, synthetic construct
  source 1..20: mol_type = other RNA
caggaacctggcacagagta

SEQ ID NO: 21962 - RNA, 20 nt, synthetic construct
  source 1..20: mol_type = other RNA
acaggaacctggcacagagt

SEQ ID NO: 21963 - RNA, 20 nt, synthetic construct
  source 1..20: mol_type = other RNA
cggaggaagggacaggaacc

SEQ ID NO: 21964 - RNA, 20 nt, synthetic construct
  source 1..20: mol_type = other RNA
tcccttcctccgtcacagca

SEQ ID NO: 21965 - RNA, 20 nt, synthetic construct
  source 1..20: mol_type = other RNA
gctgtgacggaggaagggac

SEQ ID NO: 21966 - RNA, 20 nt, synthetic construct
  source 1..20: mol_type = other RNA
accatgctgtgacggaggaa

SEQ ID NO: 21967 - RNA, 20 nt, synthetic construct
  source 1..20: mol_type = other RNA
gaccatgctgtgacggagga

SEQ ID NO: 21968 - RNA, 20 nt, synthetic construct
  source 1..20: mol_type = other RNA
cgtcacagcatggtcattcc

SEQ ID NO: 21969 - RNA, 20 nt, synthetic construct
  source 1..20: mol_type = other RNA
gaatgaccatgctgtgacgg

SEQ ID NO: 21970 - RNA, 20 nt, synthetic construct
  source 1..20: mol_type = other RNA
ctggaatgaccatgctgtga

SEQ ID NO: 21971 - RNA, 20 nt, synthetic construct
  source 1..20: mol_type = other RNA
agcatggtcattccaggata

SEQ ID NO: 21972 - RNA, 20 nt, synthetic construct
  source 1..20: mol_type = other RNA
gcatggtcattccaggatat

SEQ ID NO: 21973 - RNA, 20 nt, synthetic construct
  source 1..20: mol_type = other RNA
catggtcattccaggatatg

SEQ ID NO: 21974 - RNA, 20 nt, synthetic construct
  source 1..20: mol_type = other RNA
agtggtttgtccccatatcc

SEQ ID NO: 21975 - RNA, 20 nt, synthetic construct
  source 1..20: mol_type = other RNA
caaaccactccttcccagcc

SEQ ID NO: 21976 - RNA, 20 nt, synthetic construct
  source 1..20: mol_type = other RNA
aaaccactccttcccagcca

SEQ ID NO: 21977 - RNA, 20 nt, synthetic construct
  source 1..20: mol_type = other RNA
gcaccctggctgggaaggag

SEQ ID NO: 21978 - RNA, 20 nt, synthetic construct
  source 1..20: mol_type = other RNA
caaaggcaccctggctggga

SEQ ID NO: 21979 - RNA, 20 nt, synthetic construct
  source 1..20: mol_type = other RNA
ggctcaaaggcaccctggct

SEQ ID NO: 21980 - RNA, 20 nt, synthetic construct
  source 1..20: mol_type = other RNA
aggctcaaaggcaccctggc

SEQ ID NO: 21981 - RNA, 20 nt, synthetic construct
  source 1..20: mol_type = other RNA
gagaaggctcaaaggcaccc

SEQ ID NO: 21982 - RNA, 20 nt, synthetic construct
  source 1..20: mol_type = other RNA
ctttgagccttctcattccg

SEQ ID NO: 21983 - RNA, 20 nt, synthetic construct
  source 1..20: mol_type = other RNA
ctcggaatgagaaggctcaa

SEQ ID NO: 21984 - RNA, 20 nt, synthetic construct
  source 1..20: mol_type = other RNA
acgcagacctcggaatgaga

SEQ ID NO: 21985 - RNA, 20 nt, synthetic construct
  source 1..20: mol_type = other RNA
agggatgcaaacgcagacct

SEQ ID NO: 21986 - RNA, 20 nt, synthetic construct
  source 1..20: mol_type = other RNA
ccctgtcgtgttctccctcg

SEQ ID NO: 21987 - RNA, 20 nt, synthetic construct
  source 1..20: mol_type = other RNA
cctgtcgtgttctccctcga

SEQ ID NO: 21988 - RNA, 20 nt, synthetic construct
  source 1..20: mol_type = other RNA
ctgtcgtgttctccctcgag

SEQ ID NO: 21989 - RNA, 20 nt, synthetic construct
  source 1..20: mol_type = other RNA
cctcgagggagaacacgaca

SEQ ID NO: 21990 - RNA, 20 nt, synthetic construct
  source 1..20: mol_type = other RNA
ccctcgagggagaacacgac

SEQ ID NO: 21991 - RNA, 20 nt, synthetic construct
  source 1..20: mol_type = other RNA
gctggggaaggacccctcga

SEQ ID NO: 21992 - RNA, 20 nt, synthetic construct
  source 1..20: mol_type = other RNA
aggggtccttccccagcctg

SEQ ID NO: 21993 - RNA, 20 nt, synthetic construct
  source 1..20: mol_type = other RNA
ggggtccttccccagcctgt

SEQ ID NO: 21994 - RNA, 20 nt, synthetic construct
  source 1..20: mol_type = other RNA
gggtccttccccagcctgtg

SEQ ID NO: 21995 - RNA, 20 nt, synthetic construct
  source 1..20: mol_type = other RNA
ggtccttccccagcctgtgg

SEQ ID NO: 21996 - RNA, 20 nt, synthetic construct
  source 1..20: mol_type = other RNA
ttccccagcctgtgggggcc

SEQ ID NO: 21997 - RNA, 20 nt, synthetic construct
  source 1..20: mol_type = other RNA
tccccagcctgtgggggcct

SEQ ID NO: 21998 - RNA, 20 nt, synthetic construct
  source 1..20: mol_type = other RNA
aggcccccacaggctgggga

SEQ ID NO: 21999 - RNA, 20 nt, synthetic construct
  source 1..20: mol_type = other RNA
acccaggcccccacaggctg

SEQ ID NO: 22000 - RNA, 20 nt, synthetic construct
  source 1..20: mol_type = other RNA
gacccaggcccccacaggct

SEQ ID NO: 22001 - RNA, 20 nt, synthetic construct
  source 1..20: mol_type = other RNA
agacccaggcccccacaggc

SEQ ID NO: 22002 - RNA, 20 nt, synthetic construct
  source 1..20: mol_type = other RNA
gaacagacccaggcccccac

SEQ ID NO: 22003 - RNA, 20 nt, synthetic construct
  source 1..20: mol_type = other RNA
aatcagctcagaacagaccc

SEQ ID NO: 22004 - RNA, 20 nt, synthetic construct
  source 1..20: mol_type = other RNA
ccttttctccagttctctgc

SEQ ID NO: 22005 - RNA, 20 nt, synthetic construct
  source 1..20: mol_type = other RNA
cttttctccagttctctgct

SEQ ID NO: 22006 - RNA, 20 nt, synthetic construct
  source 1..20: mol_type = other RNA
cagcagagaactggagaaaa

SEQ ID NO: 22007 - RNA, 20 nt, synthetic construct
  source 1..20: mol_type = other RNA
ccagcagagaactggagaaa

SEQ ID NO: 22008 - RNA, 20 nt, synthetic construct
  source 1..20: mol_type = other RNA
tcttcatcccagcagagaac

SEQ ID NO: 22009 - RNA, 20 nt, synthetic construct
  source 1..20: mol_type = other RNA
tctgctgggatgaagaaagt

SEQ ID NO: 22010 - RNA, 20 nt, synthetic construct
  source 1..20: mol_type = other RNA
gaagaaagttggacactcag

SEQ ID NO: 22011 - RNA, 20 nt, synthetic construct
  source 1..20: mol_type = other RNA
aagaaagttggacactcagt

SEQ ID NO: 22012 - RNA, 20 nt, synthetic construct
  source 1..20: mol_type = other RNA
cactcagtgggaccagctgc

SEQ ID NO: 22013 - RNA, 20 nt, synthetic construct
  source 1..20: mol_type = other RNA
tcagtgggaccagctgcagg

SEQ ID NO: 22014 - RNA, 20 nt, synthetic construct
  source 1..20: mol_type = other RNA
acagtgaaaccacctgcagc

SEQ ID NO: 22015 - RNA, 20 nt, synthetic construct
  source 1..20: mol_type = other RNA
gtccccatcatgcctctcaa

SEQ ID NO: 22016 - RNA, 20 nt, synthetic construct
  source 1..20: mol_type = other RNA
tccccatcatgcctctcaat

SEQ ID NO: 22017 - RNA, 20 nt, synthetic construct
  source 1..20: mol_type = other RNA
ccccatcatgcctctcaatg

SEQ ID NO: 22018 - RNA, 20 nt, synthetic construct
  source 1..20: mol_type = other RNA
ccccattgagaggcatgatg

SEQ ID NO: 22019 - RNA, 20 nt, synthetic construct
  source 1..20: mol_type = other RNA
gccccattgagaggcatgat

SEQ ID NO: 22020 - RNA, 20 nt, synthetic construct
  source 1..20: mol_type = other RNA
ggccccattgagaggcatga

SEQ ID NO: 22021 - RNA, 20 nt, synthetic construct
  source 1..20: mol_type = other RNA
ctcaatggggcctgcaagcc

SEQ ID NO: 22022 - RNA, 20 nt, synthetic construct
  source 1..20: mol_type = other RNA
tcaatggggcctgcaagcct

SEQ ID NO: 22023 - RNA, 20 nt, synthetic construct
  source 1..20: mol_type = other RNA
ggcttgcaggccccattgag

SEQ ID NO: 22024 - RNA, 20 nt, synthetic construct
  source 1..20: mol_type = other RNA
ggcctgcaagcctgggaact

SEQ ID NO: 22025 - RNA, 20 nt, synthetic construct
  source 1..20: mol_type = other RNA
gcctgcaagcctgggaactt

SEQ ID NO: 22026 - RNA, 20 nt, synthetic construct
  source 1..20: mol_type = other RNA
gcccaagttcccaggcttgc

SEQ ID NO: 22027 - RNA, 20 nt, synthetic construct
  source 1..20: mol_type = other RNA
cctgggaacttgggcatcgt

SEQ ID NO: 22028 - RNA, 20 nt, synthetic construct
  source 1..20: mol_type = other RNA
ctgggaacttgggcatcgtt

SEQ ID NO: 22029 - RNA, 20 nt, synthetic construct
  source 1..20: mol_type = other RNA
ccaacgatgcccaagttccc

SEQ ID NO: 22030 - RNA, 20 nt, synthetic construct
  source 1..20: mol_type = other RNA
ttgggcatcgttgggccagc

SEQ ID NO: 22031 - RNA, 20 nt, synthetic construct
  source 1..20: mol_type = other RNA
gccagcaggatgagcagcaa

SEQ ID NO: 22032 - RNA, 20 nt, synthetic construct
  source 1..20: mol_type = other RNA
ccagcaggatgagcagcaaa

SEQ ID NO: 22033 - RNA, 20 nt, synthetic construct
  source 1..20: mol_type = other RNA
ccctttgctgctcatcctgc

SEQ ID NO: 22034 - RNA, 20 nt, synthetic construct
  source 1..20: mol_type = other RNA
gatgagcagcaaagggtctg

SEQ ID NO: 22035 - RNA, 20 nt, synthetic construct
  source 1..20: mol_type = other RNA
gcagcaaagggtctgaggac

SEQ ID NO: 22036 - RNA, 20 nt, synthetic construct
  source 1..20: mol_type = other RNA
cagcaaagggtctgaggaca

SEQ ID NO: 22037 - RNA, 20 nt, synthetic construct
  source 1..20: mol_type = other RNA
caaagggtctgaggacaggg

SEQ ID NO: 22038 - RNA, 20 nt, synthetic construct
  source 1..20: mol_type = other RNA
atgaagacatgcccacgcca

SEQ ID NO: 22039 - RNA, 20 nt, synthetic construct
  source 1..20: mol_type = other RNA
catgcccacgccatggagcc

SEQ ID NO: 22040 - RNA, 20 nt, synthetic construct
  source 1..20: mol_type = other RNA
atgcccacgccatggagcca

SEQ ID NO: 22041 - RNA, 20 nt, synthetic construct
  source 1..20: mol_type = other RNA
tgcccacgccatggagccag

SEQ ID NO: 22042 - RNA, 20 nt, synthetic construct
  source 1..20: mol_type = other RNA
agcccctggctccatggcgt

SEQ ID NO: 22043 - RNA, 20 nt, synthetic construct
  source 1..20: mol_type = other RNA
aagcccctggctccatggcg

SEQ ID NO: 22044 - RNA, 20 nt, synthetic construct
  source 1..20: mol_type = other RNA
ggagccaggggcttatagag

SEQ ID NO: 22045 - RNA, 20 nt, synthetic construct
  source 1..20: mol_type = other RNA
tctataagcccctggctcca

SEQ ID NO: 22046 - RNA, 20 nt, synthetic construct
  source 1..20: mol_type = other RNA
agccaggggcttatagagag

SEQ ID NO: 22047 - RNA, 20 nt, synthetic construct
  source 1..20: mol_type = other RNA
tgcccctctctataagcccc

SEQ ID NO: 22048 - RNA, 20 nt, synthetic construct
  source 1..20: mol_type = other RNA
cagagtcccatccgtcagtg

SEQ ID NO: 22049 - RNA, 20 nt, synthetic construct
  source 1..20: mol_type = other RNA
agagtcccatccgtcagtga

SEQ ID NO: 22050 - RNA, 20 nt, synthetic construct
  source 1..20: mol_type = other RNA
gagtcccatccgtcagtgag

SEQ ID NO: 22051 - RNA, 20 nt, synthetic construct
  source 1..20: mol_type = other RNA
ctcactgacggatgggactc

SEQ ID NO: 22052 - RNA, 20 nt, synthetic construct
  source 1..20: mol_type = other RNA
ccatccgtcagtgaggggac

SEQ ID NO: 22053 - RNA, 20 nt, synthetic construct
  source 1..20: mol_type = other RNA
catccgtcagtgaggggact

SEQ ID NO: 22054 - RNA, 20 nt, synthetic construct
  source 1..20: mol_type = other RNA
cagtcccctcactgacggat

SEQ ID NO: 22055 - RNA, 20 nt, synthetic construct
  source 1..20: mol_type = other RNA
ccagtcccctcactgacgga

SEQ ID NO: 22056 - RNA, 20 nt, synthetic construct
  source 1..20: mol_type = other RNA
tcagtgaggggactgggctg

SEQ ID NO: 22057 - RNA, 20 nt, synthetic construct
  source 1..20: mol_type = other RNA
cagtgaggggactgggctgc

SEQ ID NO: 22058 - RNA, 20 nt, synthetic construct
  source 1..20: mol_type = other RNA
cagcccagtcccctcactga

SEQ ID NO: 22059 - RNA, 20 nt, synthetic construct
  source 1..20: mol_type = other RNA
gaggggactgggctgcggga

SEQ ID NO: 22060 - RNA, 20 nt, synthetic construct
  source 1..20: mol_type = other RNA
aggggactgggctgcgggat

SEQ ID NO: 22061 - RNA, 20 nt, synthetic construct
  source 1..20: mol_type = other RNA
actgggctgcgggatgggtg

SEQ ID NO: 22062 - RNA, 20 nt, synthetic construct
  source 1..20: mol_type = other RNA
gtgaggatcttacagctccc

SEQ ID NO: 22063 - RNA, 20 nt, synthetic construct
  source 1..20: mol_type = other RNA
gatcttacagctcccaggtt

SEQ ID NO: 22064 - RNA, 20 nt, synthetic construct
  source 1..20: mol_type = other RNA
ggttcggaaatctaccctct

SEQ ID NO: 22065 - RNA, 20 nt, synthetic construct
  source 1..20: mol_type = other RNA
gagggtagatttccgaacct

SEQ ID NO: 22066 - RNA, 20 nt, synthetic construct
  source 1..20: mol_type = other RNA
agagggtagatttccgaacc

SEQ ID NO: 22067 - RNA, 20 nt, synthetic construct
  source 1..20: mol_type = other RNA
ggaaatctaccctctaggcc

SEQ ID NO: 22068 - RNA, 20 nt, synthetic construct
  source 1..20: mol_type = other RNA
aatctaccctctaggcctgg

SEQ ID NO: 22069 - RNA, 20 nt, synthetic construct
  source 1..20: mol_type = other RNA
gagaggcctccaggcctaga

SEQ ID NO: 22070 - RNA, 20 nt, synthetic construct
  source 1..20: mol_type = other RNA
agagaggcctccaggcctag

SEQ ID NO: 22071 - RNA, 20 nt, synthetic construct
  source 1..20: mol_type = other RNA
gaggcctctctcgcagagca

SEQ ID NO: 22072 - RNA, 20 nt, synthetic construct
  source 1..20: mol_type = other RNA
gctctgcgagagaggcctcc

SEQ ID NO: 22073 - RNA, 20 nt, synthetic construct
  source 1..20: mol_type = other RNA
cctctctcgcagagcatgga

SEQ ID NO: 22074 - RNA, 20 nt, synthetic construct
  source 1..20: mol_type = other RNA
tctcgcagagcatggaaggc

SEQ ID NO: 22075 - RNA, 20 nt, synthetic construct
  source 1..20: mol_type = other RNA
ccttccatgctctgcgagag

SEQ ID NO: 22076 - RNA, 20 nt, synthetic construct
  source 1..20: mol_type = other RNA
cagagcatggaaggcaggag

SEQ ID NO: 22077 - RNA, 20 nt, synthetic construct
  source 1..20: mol_type = other RNA
agcatggaaggcaggagagg

SEQ ID NO: 22078 - RNA, 20 nt, synthetic construct
  source 1..20: mol_type = other RNA
gcatggaaggcaggagaggt

SEQ ID NO: 22079 - RNA, 20 nt, synthetic construct
  source 1..20: mol_type = other RNA
ggaaggcaggagaggtgggc

SEQ ID NO: 22080 - RNA, 20 nt, synthetic construct
  source 1..20: mol_type = other RNA
caggagaggtgggctggcct

SEQ ID NO: 22081 - RNA, 20 nt, synthetic construct
  source 1..20: mol_type = other RNA
aggagaggtgggctggccta

SEQ ID NO: 22082 - RNA, 20 nt, synthetic construct
  source 1..20: mol_type = other RNA
gaggtgggctggcctagggc

SEQ ID NO: 22083 - RNA, 20 nt, synthetic construct
  source 1..20: mol_type = other RNA
agaagtggagctcctgccct

SEQ ID NO: 22084 - RNA, 20 nt, synthetic construct
  source 1..20: mol_type = other RNA
gctccacttctctctgcctc

SEQ ID NO: 22085 - RNA, 20 nt, synthetic construct
  source 1..20: mol_type = other RNA
cttctctctgcctctggcta

SEQ ID NO: 22086 - RNA, 20 nt, synthetic construct
  source 1..20: mol_type = other RNA
ttctctctgcctctggctat

SEQ ID NO: 22087 - RNA, 20 nt, synthetic construct
  source 1..20: mol_type = other RNA
tagccagaggcagagagaag

SEQ ID NO: 22088 - RNA, 20 nt, synthetic construct
  source 1..20: mol_type = other RNA
ctctgcctctggctatggga

SEQ ID NO: 22089 - RNA, 20 nt, synthetic construct
  source 1..20: mol_type = other RNA
ctctggctatgggaaggagc

SEQ ID NO: 22090 - RNA, 20 nt, synthetic construct
  source 1..20: mol_type = other RNA
tggctatgggaaggagcagg

SEQ ID NO: 22091 - RNA, 20 nt, synthetic construct
  source 1..20: mol_type = other RNA
ctgctccttcccatagccag

SEQ ID NO: 22092 - RNA, 20 nt, synthetic construct
  source 1..20: mol_type = other RNA
tatgggaaggagcaggcggt

SEQ ID NO: 22093 - RNA, 20 nt, synthetic construct
  source 1..20: mol_type = other RNA
ctgtgacagcagagatcttc

SEQ ID NO: 22094 - RNA, 20 nt, synthetic construct
  source 1..20: mol_type = other RNA
cagaagatctctgctgtcac

SEQ ID NO: 22095 - RNA, 20 nt, synthetic construct
  source 1..20: mol_type = other RNA
agatcttctggatttttgcc

SEQ ID NO: 22096 - RNA, 20 nt, synthetic construct
  source 1..20: mol_type = other RNA
cctggacccttctgcaagcc

SEQ ID NO: 22097 - RNA, 20 nt, synthetic construct
  source 1..20: mol_type = other RNA
ccaggcttgcagaagggtcc

SEQ ID NO: 22098 - RNA, 20 nt, synthetic construct
  source 1..20: mol_type = other RNA
ccttctgcaagcctggagac

SEQ ID NO: 22099 - RNA, 20 nt, synthetic construct
  source 1..20: mol_type = other RNA
cagtctccaggcttgcagaa

SEQ ID NO: 22100 - RNA, 20 nt, synthetic construct
  source 1..20: mol_type = other RNA
ccagtctccaggcttgcaga

SEQ ID NO: 22101 - RNA, 20 nt, synthetic construct
  source 1..20: mol_type = other RNA
atgtggcaggtccagtctcc

SEQ ID NO: 22102 - RNA, 20 nt, synthetic construct
  source 1..20: mol_type = other RNA
acagacttggaacatgtggc

SEQ ID NO: 22103 - RNA, 20 nt, synthetic construct
  source 1..20: mol_type = other RNA
gcagacagacttggaacatg

SEQ ID NO: 22104 - RNA, 20 nt, synthetic construct
  source 1..20: mol_type = other RNA
gtgacctaggcagacagact

SEQ ID NO: 22105 - RNA, 20 nt, synthetic construct
  source 1..20: mol_type = other RNA
agaagtggcagcagtgacct

SEQ ID NO: 22106 - RNA, 20 nt, synthetic construct
  source 1..20: mol_type = other RNA
tctgttagtgggaggagaag

SEQ ID NO: 22107 - RNA, 20 nt, synthetic construct
  source 1..20: mol_type = other RNA
aagaaaggtctgttagtggg

SEQ ID NO: 22108 - RNA, 20 nt, synthetic construct
  source 1..20: mol_type = other RNA
ttcaagaaaggtctgttagt

SEQ ID NO: 22109 - RNA, 20 nt, synthetic construct
  source 1..20: mol_type = other RNA
cttcaagaaaggtctgttag

SEQ ID NO: 22110 - RNA, 20 nt, synthetic construct
  source 1..20: mol_type = other RNA
acctttcttgaagacccact

SEQ ID NO: 22111 - RNA, 20 nt, synthetic construct
  source 1..20: mol_type = other RNA
acctagtgggtcttcaagaa

SEQ ID NO: 22112 - RNA, 20 nt, synthetic construct
  source 1..20: mol_type = other RNA
ccactaggtccagacactgc

SEQ ID NO: 22113 - RNA, 20 nt, synthetic construct
  source 1..20: mol_type = other RNA
cactaggtccagacactgcc

SEQ ID NO: 22114 - RNA, 20 nt, synthetic construct
  source 1..20: mol_type = other RNA
cggcagtgtctggacctagt

SEQ ID NO: 22115 - RNA, 20 nt, synthetic construct
  source 1..20: mol_type = other RNA
ccggcagtgtctggacctag

SEQ ID NO: 22116 - RNA, 20 nt, synthetic construct
  source 1..20: mol_type = other RNA
cagacactgccgggacttgc

SEQ ID NO: 22117 - RNA, 20 nt, synthetic construct
  source 1..20: mol_type = other RNA
ctgcaagtcccggcagtgtc

SEQ ID NO: 22118 - RNA, 20 nt, synthetic construct
  source 1..20: mol_type = other RNA
actgccgggacttgcaggta

SEQ ID NO: 22119 - RNA, 20 nt, synthetic construct
  source 1..20: mol_type = other RNA
ctgccgggacttgcaggtat

SEQ ID NO: 22120 - RNA, 20 nt, synthetic construct
  source 1..20: mol_type = other RNA
tgccgggacttgcaggtatg

SEQ ID NO: 22121 - RNA, 20 nt, synthetic construct
  source 1..20: mol_type = other RNA
gccgggacttgcaggtatgg

SEQ ID NO: 22122 - RNA, 20 nt, synthetic construct
  source 1..20: mol_type = other RNA
ccgggacttgcaggtatggg

SEQ ID NO: 22123 - RNA, 20 nt, synthetic construct
  source 1..20: mol_type = other RNA
ccccccatacctgcaagtcc

SEQ ID NO: 22124 - RNA, 20 nt, synthetic construct
  source 1..20: mol_type = other RNA
ttgcaggtatggggggtaga

SEQ ID NO: 22125 - RNA, 20 nt, synthetic construct
  source 1..20: mol_type = other RNA
ggtatggggggtagaaggag

SEQ ID NO: 22126 - RNA, 20 nt, synthetic construct
  source 1..20: mol_type = other RNA
ggagaggcagataagctgcc

SEQ ID NO: 22127 - RNA, 20 nt, synthetic construct
  source 1..20: mol_type = other RNA
gagaggcagataagctgcct

SEQ ID NO: 22128 - RNA, 20 nt, synthetic construct
  source 1..20: mol_type = other RNA
agaggcagataagctgcctg

SEQ ID NO: 22129 - RNA, 20 nt, synthetic construct
  source 1..20: mol_type = other RNA
gaggcagataagctgcctgg

SEQ ID NO: 22130 - RNA, 20 nt, synthetic construct
  source 1..20: mol_type = other RNA
aggcagataagctgcctggg

SEQ ID NO: 22131 - RNA, 20 nt, synthetic construct
  source 1..20: mol_type = other RNA
cctggggggctgttagctaa

SEQ ID NO: 22132 - RNA, 20 nt, synthetic construct
  source 1..20: mol_type = other RNA
ctggggggctgttagctaat

SEQ ID NO: 22133 - RNA, 20 nt, synthetic construct
  source 1..20: mol_type = other RNA
ccattagctaacagcccccc

SEQ ID NO: 22134 - RNA, 20 nt, synthetic construct
  source 1..20: mol_type = other RNA
gctgttagctaatgggtaca

SEQ ID NO: 22135 - RNA, 20 nt, synthetic construct
  source 1..20: mol_type = other RNA
tggcttctcttctcgggagg

SEQ ID NO: 22136 - RNA, 20 nt, synthetic construct
  source 1..20: mol_type = other RNA
gtggcttctcttctcgggag

SEQ ID NO: 22137 - RNA, 20 nt, synthetic construct
  source 1..20: mol_type = other RNA
tgtggcttctcttctcggga

SEQ ID NO: 22138 - RNA, 20 nt, synthetic construct
  source 1..20: mol_type = other RNA
ctgtggcttctcttctcggg

SEQ ID NO: 22139 - RNA, 20 nt, synthetic construct
  source 1..20: mol_type = other RNA
gaagagaagccacagatgag

SEQ ID NO: 22140 - RNA, 20 nt, synthetic construct
  source 1..20: mol_type = other RNA
aagagaagccacagatgagt

SEQ ID NO: 22141 - RNA, 20 nt, synthetic construct
  source 1..20: mol_type = other RNA
cacagatgagtgggccagcg

SEQ ID NO: 22142 - RNA, 20 nt, synthetic construct
  source 1..20: mol_type = other RNA
ctcgctggcccactcatctg

SEQ ID NO: 22143 - RNA, 20 nt, synthetic construct
  source 1..20: mol_type = other RNA
acattgaagactggcctcgc

SEQ ID NO: 22144 - RNA, 20 nt, synthetic construct
  source 1..20: mol_type = other RNA
aattagtggacattgaagac

SEQ ID NO: 22145 - RNA, 20 nt, synthetic construct
  source 1..20: mol_type = other RNA
actaattcactctaagcatt

SEQ ID NO: 22146 - RNA, 20 nt, synthetic construct
  source 1..20: mol_type = other RNA
aaatgcttagagtgaattag

SEQ ID NO: 22147 - RNA, 20 nt, synthetic construct
  source 1..20: mol_type = other RNA
ctaagcatttggccaaaaaa

SEQ ID NO: 22148 - RNA, 20 nt, synthetic construct
  source 1..20: mol_type = other RNA
ttatttctctctcctttttt

SEQ ID NO: 22149 - RNA, 20 nt, synthetic construct
  source 1..20: mol_type = other RNA
agaaataactgaaattgttc

SEQ ID NO: 22150 - RNA, 20 nt, synthetic construct
  source 1..20: mol_type = other RNA
aataactgaaattgttcagg

SEQ ID NO: 22151 - RNA, 20 nt, synthetic construct
  source 1..20: mol_type = other RNA
tggctccatcgtctattctg

SEQ ID NO: 22152 - RNA, 20 nt, synthetic construct
  source 1..20: mol_type = other RNA
ggggaccacagaatagacga

SEQ ID NO: 22153 - RNA, 20 nt, synthetic construct
  source 1..20: mol_type = other RNA
cctccatgagcctttgcccc

SEQ ID NO: 22154 - RNA, 20 nt, synthetic construct
  source 1..20: mol_type = other RNA
ctccatgagcctttgcccca

SEQ ID NO: 22155 - RNA, 20 nt, synthetic construct
  source 1..20: mol_type = other RNA
tggggcaaaggctcatggag

SEQ ID NO: 22156 - RNA, 20 nt, synthetic construct
  source 1..20: mol_type = other RNA
catgagcctttgccccaggg

SEQ ID NO: 22157 - RNA, 20 nt, synthetic construct
  source 1..20: mol_type = other RNA
cctggggcaaaggctcatgg

SEQ ID NO: 22158 - RNA, 20 nt, synthetic construct
  source 1..20: mol_type = other RNA
caccctggggcaaaggctca

SEQ ID NO: 22159 - RNA, 20 nt, synthetic construct
  source 1..20: mol_type = other RNA
ctttgccccagggtgggtgc

SEQ ID NO: 22160 - RNA, 20 nt, synthetic construct
  source 1..20: mol_type = other RNA
ctgcacccaccctggggcaa

SEQ ID NO: 22161 - RNA, 20 nt, synthetic construct
  source 1..20: mol_type = other RNA
tcgcacctgcacccaccctg

SEQ ID NO: 22162 - RNA, 20 nt, synthetic construct
  source 1..20: mol_type = other RNA
ctcgcacctgcacccaccct

SEQ ID NO: 22163 - RNA, 20 nt, synthetic construct
  source 1..20: mol_type = other RNA
actcgcacctgcacccaccc

SEQ ID NO: 22164 - RNA, 20 nt, synthetic construct
  source 1..20: mol_type = other RNA
tgaatgactgaggcagctgc

SEQ ID NO: 22165 - RNA, 20 nt, synthetic construct
  source 1..20: mol_type = other RNA
tctggaactctgaatgactg

SEQ ID NO: 22166 - RNA, 20 nt, synthetic construct
  source 1..20: mol_type = other RNA
cagagttccagagccttctg

SEQ ID NO: 22167 - RNA, 20 nt, synthetic construct
  source 1..20: mol_type = other RNA
agttccagagccttctgtgg

SEQ ID NO: 22168 - RNA, 20 nt, synthetic construct
  source 1..20: mol_type = other RNA
tgctccaccacagaaggctc

SEQ ID NO: 22169 - RNA, 20 nt, synthetic construct
  source 1..20: mol_type = other RNA
gcaggatgctccaccacaga

SEQ ID NO: 22170 - RNA, 20 nt, synthetic construct
  source 1..20: mol_type = other RNA
tggtggagcatcctgctgct

SEQ ID NO: 22171 - RNA, 20 nt, synthetic construct
  source 1..20: mol_type = other RNA
tggagcatcctgctgcttgg

SEQ ID NO: 22172 - RNA, 20 nt, synthetic construct
  source 1..20: mol_type = other RNA
agactcatcctccaagcagc

SEQ ID NO: 22173 - RNA, 20 nt, synthetic construct
  source 1..20: mol_type = other RNA
atgagtctgaagtttaaaaa

SEQ ID NO: 22174 - RNA, 20 nt, synthetic construct
  source 1..20: mol_type = other RNA
tgagtctgaagtttaaaaat

SEQ ID NO: 22175 - RNA, 20 nt, synthetic construct
  source 1..20: mol_type = other RNA
tcatcaggggggctcagaaa

SEQ ID NO: 22176 - RNA, 20 nt, synthetic construct
  source 1..20: mol_type = other RNA
gcactgactgctcatcaggg

SEQ ID NO: 22177 - RNA, 20 nt, synthetic construct
  source 1..20: mol_type = other RNA
agcactgactgctcatcagg

SEQ ID NO: 22178 - RNA, 20 nt, synthetic construct
  source 1..20: mol_type = other RNA
aagcactgactgctcatcag

SEQ ID NO: 22179 - RNA, 20 nt, synthetic construct
  source 1..20: mol_type = other RNA
gaagcactgactgctcatca

SEQ ID NO: 22180 - RNA, 20 nt, synthetic construct
  source 1..20: mol_type = other RNA
agaagcactgactgctcatc

SEQ ID NO: 22181 - RNA, 20 nt, synthetic construct
  source 1..20: mol_type = other RNA
agtgcttctgggcccagcta

SEQ ID NO: 22182 - RNA, 20 nt, synthetic construct
  source 1..20: mol_type = other RNA
aacagatggcttccttagct

SEQ ID NO: 22183 - RNA, 20 nt, synthetic construct
  source 1..20: mol_type = other RNA
gaacagatggcttccttagc

SEQ ID NO: 22184 - RNA, 20 nt, synthetic construct
  source 1..20: mol_type = other RNA
aagccatctgttcccagcag

SEQ ID NO: 22185 - RNA, 20 nt, synthetic construct
  source 1..20: mol_type = other RNA
tctcctctgctgggaacaga

SEQ ID NO: 22186 - RNA, 20 nt, synthetic construct
  source 1..20: mol_type = other RNA
cgcagcagctctcctctgct

SEQ ID NO: 22187 - RNA, 20 nt, synthetic construct
  source 1..20: mol_type = other RNA
gcgcagcagctctcctctgc

SEQ ID NO: 22188 - RNA, 20 nt, synthetic construct
  source 1..20: mol_type = other RNA
gctgctgcgctgacctgcag

SEQ ID NO: 22189 - RNA, 20 nt, synthetic construct
  source 1..20: mol_type = other RNA
ctgcgctgacctgcagaggt

SEQ ID NO: 22190 - RNA, 20 nt, synthetic construct
  source 1..20: mol_type = other RNA
cgctgacctgcagaggttgg

SEQ ID NO: 22191 - RNA, 20 nt, synthetic construct
  source 1..20: mol_type = other RNA
ctgggaccaccaacctctgc

SEQ ID NO: 22192 - RNA, 20 nt, synthetic construct
  source 1..20: mol_type = other RNA
ccagcacagagctgtgccca

SEQ ID NO: 22193 - RNA, 20 nt, synthetic construct
  source 1..20: mol_type = other RNA
cagcacagagctgtgcccat

SEQ ID NO: 22194 - RNA, 20 nt, synthetic construct
  source 1..20: mol_type = other RNA
catgggcacagctctgtgct

SEQ ID NO: 22195 - RNA, 20 nt, synthetic construct
  source 1..20: mol_type = other RNA
ccatgggcacagctctgtgc

SEQ ID NO: 22196 - RNA, 20 nt, synthetic construct
  source 1..20: mol_type = other RNA
tgtgcccatgggcttgttag

SEQ ID NO: 22197 - RNA, 20 nt, synthetic construct
  source 1..20: mol_type = other RNA
gtgcccatgggcttgttagt

SEQ ID NO: 22198 - RNA, 20 nt, synthetic construct
  source 1..20: mol_type = other RNA
tttcccactaacaagcccat

SEQ ID NO: 22199 - RNA, 20 nt, synthetic construct
  source 1..20: mol_type = other RNA
ttttcccactaacaagccca

SEQ ID NO: 22200 - RNA, 20 nt, synthetic construct
  source 1..20: mol_type = other RNA
ggcattcataattaaatgtt

SEQ ID NO: 22201 - RNA, 20 nt, synthetic construct
  source 1..20: mol_type = other RNA
agatctagatgctggggagt

SEQ ID NO: 22202 - RNA, 20 nt, synthetic construct
  source 1..20: mol_type = other RNA
tagatctagatgctggggag

SEQ ID NO: 22203 - RNA, 20 nt, synthetic construct
  source 1..20: mol_type = other RNA
aattttagatctagatgctg

SEQ ID NO: 22204 - RNA, 20 nt, synthetic construct
  source 1..20: mol_type = other RNA
taattttagatctagatgct

SEQ ID NO: 22205 - RNA, 20 nt, synthetic construct
  source 1..20: mol_type = other RNA
ataattttagatctagatgc

SEQ ID NO: 22206 - RNA, 20 nt, synthetic construct
  source 1..20: mol_type = other RNA
acagagagagaaaaagaatg

SEQ ID NO: 22207 - RNA, 20 nt, synthetic construct
  source 1..20: mol_type = other RNA
ttgcaatgtacttttaaatt

SEQ ID NO: 22208 - RNA, 20 nt, synthetic construct
  source 1..20: mol_type = other RNA
gatgcaggctgaagctttca

SEQ ID NO: 22209 - RNA, 20 nt, synthetic construct
  source 1..20: mol_type = other RNA
agatgcaggctgaagctttc

SEQ ID NO: 22210 - RNA, 20 nt, synthetic construct
  source 1..20: mol_type = other RNA
gcctgcatctcctaagagtt

SEQ ID NO: 22211 - RNA, 20 nt, synthetic construct
  source 1..20: mol_type = other RNA
cctgcatctcctaagagtta

SEQ ID NO: 22212 - RNA, 20 nt, synthetic construct
  source 1..20: mol_type = other RNA
ccctaactcttaggagatgc

SEQ ID NO: 22213 - RNA, 20 nt, synthetic construct
  source 1..20: mol_type = other RNA
aggacaatgccctaactctt

SEQ ID NO: 22214 - RNA, 20 nt, synthetic construct
  source 1..20: mol_type = other RNA
tagggcattgtcctacacat

SEQ ID NO: 22215 - RNA, 20 nt, synthetic construct
  source 1..20: mol_type = other RNA
gtgatactgggccaatgtgt

SEQ ID NO: 22216 - RNA, 20 nt, synthetic construct
  source 1..20: mol_type = other RNA
ctcgtcttggctgtgatact

SEQ ID NO: 22217 - RNA, 20 nt, synthetic construct
  source 1..20: mol_type = other RNA
tctcgtcttggctgtgatac

SEQ ID NO: 22218 - RNA, 20 nt, synthetic construct
  source 1..20: mol_type = other RNA
tgggaaatgacttctcgtct

SEQ ID NO: 22219 - RNA, 20 nt, synthetic construct
  source 1..20: mol_type = other RNA
attagatagcagacatcgct

SEQ ID NO: 22220 - RNA, 20 nt, synthetic construct
  source 1..20: mol_type = other RNA
gattagatagcagacatcgc

SEQ ID NO: 22221 - RNA, 20 nt, synthetic construct
  source 1..20: mol_type = other RNA
aatccccccaattgtctccc

SEQ ID NO: 22222 - RNA, 20 nt, synthetic construct
  source 1..20: mol_type = other RNA
ttacctgggagacaattggg

SEQ ID NO: 22223 - RNA, 20 nt, synthetic construct
  source 1..20: mol_type = other RNA
gttacctgggagacaattgg

SEQ ID NO: 22224 - RNA, 20 nt, synthetic construct
  source 1..20: mol_type = other RNA
agttacctgggagacaattg

SEQ ID NO: 22225 - RNA, 20 nt, synthetic construct
  source 1..20: mol_type = other RNA
aagttacctgggagacaatt

SEQ ID NO: 22226 - RNA, 20 nt, synthetic construct
  source 1..20: mol_type = other RNA
taagttacctgggagacaat

SEQ ID NO: 22227 - RNA, 20 nt, synthetic construct
  source 1..20: mol_type = other RNA
tcccaggtaacttatgtgtc

SEQ ID NO: 22228 - RNA, 20 nt, synthetic construct
  source 1..20: mol_type = other RNA
accagacacataagttacct

SEQ ID NO: 22229 - RNA, 20 nt, synthetic construct
  source 1..20: mol_type = other RNA
aaccagacacataagttacc

SEQ ID NO: 22230 - RNA, 20 nt, synthetic construct
  source 1..20: mol_type = other RNA
ttggaatcagcatccagtca

SEQ ID NO: 22231 - RNA, 20 nt, synthetic construct
  source 1..20: mol_type = other RNA
tgcaatgtgtgcaccgtgac

SEQ ID NO: 22232 - RNA, 20 nt, synthetic construct
  source 1..20: mol_type = other RNA
aaacctctttgaatgctgaa

SEQ ID NO: 22233 - RNA, 20 nt, synthetic construct
  source 1..20: mol_type = other RNA
agacctttcagcattcaaag

SEQ ID NO: 22234 - RNA, 20 nt, synthetic construct
  source 1..20: mol_type = other RNA
aaaaactcaaagtgagctga

SEQ ID NO: 22235 - RNA, 20 nt, synthetic construct
  source 1..20: mol_type = other RNA
taaaaactcaaagtgagctg

SEQ ID NO: 22236 - RNA, 20 nt, synthetic construct
  source 1..20: mol_type = other RNA
tttaaatgacattgtttttg

SEQ ID NO: 22237 - RNA, 20 nt, synthetic construct
  source 1..20: mol_type = other RNA
gacattgtttttgaggccct

SEQ ID NO: 22238 - RNA, 20 nt, synthetic construct
  source 1..20: mol_type = other RNA
tcaaaaagacagcaggccta

SEQ ID NO: 22239 - RNA, 20 nt, synthetic construct
  source 1..20: mol_type = other RNA
ttcaaaaagacagcaggcct

SEQ ID NO: 22240 - RNA, 20 nt, synthetic construct
  source 1..20: mol_type = other RNA
tggggcttcaaaaagacagc

SEQ ID NO: 22241 - RNA, 20 nt, synthetic construct
  source 1..20: mol_type = other RNA
tctgacaaattcagaatgtg

SEQ ID NO: 22242 - RNA, 20 nt, synthetic construct
  source 1..20: mol_type = other RNA
atctgacaaattcagaatgt

SEQ ID NO: 22243 - RNA, 20 nt, synthetic construct
  source 1..20: mol_type = other RNA
aatctgacaaattcagaatg

SEQ ID NO: 22244 - RNA, 20 nt, synthetic construct
  source 1..20: mol_type = other RNA
tttgtcagattgtttgctca

SEQ ID NO: 22245 - RNA, 20 nt, synthetic construct
  source 1..20: mol_type = other RNA
agtacaggggatagaagaag

SEQ ID NO: 22246 - RNA, 20 nt, synthetic construct
  source 1..20: mol_type = other RNA
ttctatcccctgtactttca

SEQ ID NO: 22247 - RNA, 20 nt, synthetic construct
  source 1..20: mol_type = other RNA
tgtactttcaaggataattt

SEQ ID NO: 22248 - RNA, 20 nt, synthetic construct
  source 1..20: mol_type = other RNA
aattatccttgaaagtacag

SEQ ID NO: 22249 - RNA, 20 nt, synthetic construct
  source 1..20: mol_type = other RNA
aaattatccttgaaagtaca

SEQ ID NO: 22250 - RNA, 20 nt, synthetic construct
  source 1..20: mol_type = other RNA
taaattatccttgaaagtac

SEQ ID NO: 22251 - RNA, 20 nt, synthetic construct
  source 1..20: mol_type = other RNA
agctgtcaagtcagcacaaa

SEQ ID NO: 22252 - RNA, 20 nt, synthetic construct
  source 1..20: mol_type = other RNA
tgacagtggaggcgcatctt

SEQ ID NO: 22253 - RNA, 20 nt, synthetic construct
  source 1..20: mol_type = other RNA
cttggtacaggtgacagtgg

SEQ ID NO: 22254 - RNA, 20 nt, synthetic construct
  source 1..20: mol_type = other RNA
gcacttggtacaggtgacag

SEQ ID NO: 22255 - RNA, 20 nt, synthetic construct
  source 1..20: mol_type = other RNA
accaagtgccaaaacagcag

SEQ ID NO: 22256 - RNA, 20 nt, synthetic construct
  source 1..20: mol_type = other RNA
ccaagtgccaaaacagcaga

SEQ ID NO: 22257 - RNA, 20 nt, synthetic construct
  source 1..20: mol_type = other RNA
caagtgccaaaacagcagag

SEQ ID NO: 22258 - RNA, 20 nt, synthetic construct
  source 1..20: mol_type = other RNA
ccctctgctgttttggcact

SEQ ID NO: 22259 - RNA, 20 nt, synthetic construct
  source 1..20: mol_type = other RNA
aactggcccctctgctgttt

SEQ ID NO: 22260 - RNA, 20 nt, synthetic construct
  source 1..20: mol_type = other RNA
gccagttagagcaagagctc

SEQ ID NO: 22261 - RNA, 20 nt, synthetic construct
  source 1..20: mol_type = other RNA
ccagttagagcaagagctct

SEQ ID NO: 22262 - RNA, 20 nt, synthetic construct
  source 1..20: mol_type = other RNA
cagttagagcaagagctctg

SEQ ID NO: 22263 - RNA, 20 nt, synthetic construct
  source 1..20: mol_type = other RNA
agttagagcaagagctctgg

SEQ ID NO: 22264 - RNA, 20 nt, synthetic construct
  source 1..20: mol_type = other RNA
gttagagcaagagctctggg

SEQ ID NO: 22265 - RNA, 20 nt, synthetic construct
  source 1..20: mol_type = other RNA
ttagagcaagagctctgggg

SEQ ID NO: 22266 - RNA, 20 nt, synthetic construct
  source 1..20: mol_type = other RNA
cccagagctcttgctctaac

SEQ ID NO: 22267 - RNA, 20 nt, synthetic construct
  source 1..20: mol_type = other RNA
agcaagagctctgggggggc

SEQ ID NO: 22268 - RNA, 20 nt, synthetic construct
  source 1..20: mol_type = other RNA
ggggggccggaaagtctccc

SEQ ID NO: 22269 - RNA, 20 nt, synthetic construct
  source 1..20: mol_type = other RNA
ccggaaagtctccctggaga

SEQ ID NO: 22270 - RNA, 20 nt, synthetic construct
  source 1..20: mol_type = other RNA
ccttctccagggagactttc

SEQ ID NO: 22271 - RNA, 20 nt, synthetic construct
  source 1..20: mol_type = other RNA
ctggagaaggccgtaatatc

SEQ ID NO: 22272 - RNA, 20 nt, synthetic construct
  source 1..20: mol_type = other RNA
tggagaaggccgtaatatct

SEQ ID NO: 22273 - RNA, 20 nt, synthetic construct
  source 1..20: mol_type = other RNA
agatattacggccttctcca

SEQ ID NO: 22274 - RNA, 20 nt, synthetic construct
  source 1..20: mol_type = other RNA
cagatattacggccttctcc

SEQ ID NO: 22275 - RNA, 20 nt, synthetic construct
  source 1..20: mol_type = other RNA
aggccgtaatatctgggcct

SEQ ID NO: 22276 - RNA, 20 nt, synthetic construct
  source 1..20: mol_type = other RNA
cgtaatatctgggccttgga

SEQ ID NO: 22277 - RNA, 20 nt, synthetic construct
  source 1..20: mol_type = other RNA
atatctgggccttggaagga

SEQ ID NO: 22278 - RNA, 20 nt, synthetic construct
  source 1..20: mol_type = other RNA
ggccttggaaggaaggacac

SEQ ID NO: 22279 - RNA, 20 nt, synthetic construct
  source 1..20: mol_type = other RNA
gccttggaaggaaggacaca

SEQ ID NO: 22280 - RNA, 20 nt, synthetic construct
  source 1..20: mol_type = other RNA
gccctgtgtccttccttcca

SEQ ID NO: 22281 - RNA, 20 nt, synthetic construct
  source 1..20: mol_type = other RNA
gaaggacacagggctctgga

SEQ ID NO: 22282 - RNA, 20 nt, synthetic construct
  source 1..20: mol_type = other RNA
ggacacagggctctggaagg

SEQ ID NO: 22283 - RNA, 20 nt, synthetic construct
  source 1..20: mol_type = other RNA
cacagggctctggaaggagg

SEQ ID NO: 22284 - RNA, 20 nt, synthetic construct
  source 1..20: mol_type = other RNA
ggaggaggctgcatgcctga

SEQ ID NO: 22285 - RNA, 20 nt, synthetic construct
  source 1..20: mol_type = other RNA
gaggctgcatgcctgaaggc

SEQ ID NO: 22286 - RNA, 20 nt, synthetic construct
  source 1..20: mol_type = other RNA
aggctgcatgcctgaaggct

SEQ ID NO: 22287 - RNA, 20 nt, synthetic construct
  source 1..20: mol_type = other RNA
gaaggctgggccttcgaccc

SEQ ID NO: 22288 - RNA, 20 nt, synthetic construct
  source 1..20: mol_type = other RNA
aaggctgggccttcgaccct

SEQ ID NO: 22289 - RNA, 20 nt, synthetic construct
  source 1..20: mol_type = other RNA
aggctgggccttcgaccctg

SEQ ID NO: 22290 - RNA, 20 nt, synthetic construct
  source 1..20: mol_type = other RNA
tgggccttcgaccctgggga

SEQ ID NO: 22291 - RNA, 20 nt, synthetic construct
  source 1..20: mol_type = other RNA
gggccttcgaccctggggat

SEQ ID NO: 22292 - RNA, 20 nt, synthetic construct
  source 1..20: mol_type = other RNA
cgaccctggggatgggccac

SEQ ID NO: 22293 - RNA, 20 nt, synthetic construct
  source 1..20: mol_type = other RNA
gaccctggggatgggccaca

SEQ ID NO: 22294 - RNA, 20 nt, synthetic construct
  source 1..20: mol_type = other RNA
tgccctgtggcccatcccca

SEQ ID NO: 22295 - RNA, 20 nt, synthetic construct
  source 1..20: mol_type = other RNA
gtgccctgtggcccatcccc

SEQ ID NO: 22296 - RNA, 20 nt, synthetic construct
  source 1..20: mol_type = other RNA
atgatgtgtttggtgccctg

SEQ ID NO: 22297 - RNA, 20 nt, synthetic construct
  source 1..20: mol_type = other RNA
agagagacatatgatgtgtt

SEQ ID NO: 22298 - RNA, 20 nt, synthetic construct
  source 1..20: mol_type = other RNA
atgtctctctctttctattt

SEQ ID NO: 22299 - RNA, 20 nt, synthetic construct
  source 1..20: mol_type = other RNA
tgtctctctctttctatttt

SEQ ID NO: 22300 - RNA, 20 nt, synthetic construct
  source 1..20: mol_type = other RNA
gtctctctctttctattttg

SEQ ID NO: 22301 - RNA, 20 nt, synthetic construct
  source 1..20: mol_type = other RNA
tctttctattttggggtccc

SEQ ID NO: 22302 - RNA, 20 nt, synthetic construct
  source 1..20: mol_type = other RNA
ctttctattttggggtccca

SEQ ID NO: 22303 - RNA, 20 nt, synthetic construct
  source 1..20: mol_type = other RNA
gtcccagggttttcatttcc

SEQ ID NO: 22304 - RNA, 20 nt, synthetic construct
  source 1..20: mol_type = other RNA
ctccaggaaatgaaaaccct

SEQ ID NO: 22305 - RNA, 20 nt, synthetic construct
  source 1..20: mol_type = other RNA
tctccaggaaatgaaaaccc

SEQ ID NO: 22306 - RNA, 20 nt, synthetic construct
  source 1..20: mol_type = other RNA
tttcatttcctggagacccg

SEQ ID NO: 22307 - RNA, 20 nt, synthetic construct
  source 1..20: mol_type = other RNA
cacacagaccacgggtctcc

SEQ ID NO: 22308 - RNA, 20 nt, synthetic construct
  source 1..20: mol_type = other RNA
gacccgtggtctgtgtgcac

SEQ ID NO: 22309 - RNA, 20 nt, synthetic construct
  source 1..20: mol_type = other RNA
ctccagtgcacacagaccac

SEQ ID NO: 22310 - RNA, 20 nt, synthetic construct
  source 1..20: mol_type = other RNA
gctccagtgcacacagacca

SEQ ID NO: 22311 - RNA, 20 nt, synthetic construct
  source 1..20: mol_type = other RNA
gtgtgcactggagcagagcc

SEQ ID NO: 22312 - RNA, 20 nt, synthetic construct
  source 1..20: mol_type = other RNA
gccaggctctcagttgcagc

SEQ ID NO: 22313 - RNA, 20 nt, synthetic construct
  source 1..20: mol_type = other RNA
ccaggctctcagttgcagca

SEQ ID NO: 22314 - RNA, 20 nt, synthetic construct
  source 1..20: mol_type = other RNA
ccctgctgcaactgagagcc

SEQ ID NO: 22315 - RNA, 20 nt, synthetic construct
  source 1..20: mol_type = other RNA
gcagcagggaaaagcctaca

SEQ ID NO: 22316 - RNA, 20 nt, synthetic construct
  source 1..20: mol_type = other RNA
cagcagggaaaagcctacat

SEQ ID NO: 22317 - RNA, 20 nt, synthetic construct
  source 1..20: mol_type = other RNA
agcagggaaaagcctacatg

SEQ ID NO: 22318 - RNA, 20 nt, synthetic construct
  source 1..20: mol_type = other RNA
cgggaggcagttccccatgt

SEQ ID NO: 22319 - RNA, 20 nt, synthetic construct
  source 1..20: mol_type = other RNA
gaactgcctcccgcaagctg

SEQ ID NO: 22320 - RNA, 20 nt, synthetic construct
  source 1..20: mol_type = other RNA
ctcacaccacagcttgcggg

SEQ ID NO: 22321 - RNA, 20 nt, synthetic construct
  source 1..20: mol_type = other RNA
cttctcacaccacagcttgc

SEQ ID NO: 22322 - RNA, 20 nt, synthetic construct
  source 1..20: mol_type = other RNA
tcttctcacaccacagcttg

SEQ ID NO: 22323 - RNA, 20 nt, synthetic construct
  source 1..20: mol_type = other RNA
ctgtggtgtgagaagagccc

SEQ ID NO: 22324 - RNA, 20 nt, synthetic construct
  source 1..20: mol_type = other RNA
ggtgtgagaagagccctggc

SEQ ID NO: 22325 - RNA, 20 nt, synthetic construct
  source 1..20: mol_type = other RNA
gaagagccctggctggcagc

SEQ ID NO: 22326 - RNA, 20 nt, synthetic construct
  source 1..20: mol_type = other RNA
acagctcctgctgccagcca

SEQ ID NO: 22327 - RNA, 20 nt, synthetic construct
  source 1..20: mol_type = other RNA
cacagctcctgctgccagcc

SEQ ID NO: 22328 - RNA, 20 nt, synthetic construct
  source 1..20: mol_type = other RNA
ctgtgaagtttcatcccagc

SEQ ID NO: 22329 - RNA, 20 nt, synthetic construct
  source 1..20: mol_type = other RNA
tgtgaagtttcatcccagcc

SEQ ID NO: 22330 - RNA, 20 nt, synthetic construct
  source 1..20: mol_type = other RNA
gctactaaatgcacccggct

SEQ ID NO: 22331 - RNA, 20 nt, synthetic construct
  source 1..20: mol_type = other RNA
agctactaaatgcacccggc

SEQ ID NO: 22332 - RNA, 20 nt, synthetic construct
  source 1..20: mol_type = other RNA
aggcagctactaaatgcacc

SEQ ID NO: 22333 - RNA, 20 nt, synthetic construct
  source 1..20: mol_type = other RNA
tgcctgaccatcttcctccc

SEQ ID NO: 22334 - RNA, 20 nt, synthetic construct
  source 1..20: mol_type = other RNA
ggcctgggaggaagatggtc

SEQ ID NO: 22335 - RNA, 20 nt, synthetic construct
  source 1..20: mol_type = other RNA
ctgagggcctgggaggaaga

SEQ ID NO: 22336 - RNA, 20 nt, synthetic construct
  source 1..20: mol_type = other RNA
gaagaaactgagggcctggg

SEQ ID NO: 22337 - RNA, 20 nt, synthetic construct
  source 1..20: mol_type = other RNA
gatgaagaaactgagggcct

SEQ ID NO: 22338 - RNA, 20 nt, synthetic construct
  source 1..20: mol_type = other RNA
agatgaagaaactgagggcc

SEQ ID NO: 22339 - RNA, 20 nt, synthetic construct
  source 1..20: mol_type = other RNA
tctacagatgaagaaactga

SEQ ID NO: 22340 - RNA, 20 nt, synthetic construct
  source 1..20: mol_type = other RNA
ttctacagatgaagaaactg

SEQ ID NO: 22341 - RNA, 20 nt, synthetic construct
  source 1..20: mol_type = other RNA
catctgtagaatgagcagat

SEQ ID NO: 22342 - RNA, 20 nt, synthetic construct
  source 1..20: mol_type = other RNA
atctgtagaatgagcagata

SEQ ID NO: 22343 - RNA, 20 nt, synthetic construct
  source 1..20: mol_type = other RNA
tctgtagaatgagcagatag

SEQ ID NO: 22344 - RNA, 20 nt, synthetic construct
  source 1..20: mol_type = other RNA
gagcagataggggccacagc

SEQ ID NO: 22345 - RNA, 20 nt, synthetic construct
  source 1..20: mol_type = other RNA
agcagataggggccacagca

SEQ ID NO: 22346 - RNA, 20 nt, synthetic construct
  source 1..20: mol_type = other RNA
atgtgtgaaaatccctgctg

SEQ ID NO: 22347 - RNA, 20 nt, synthetic construct
  source 1..20: mol_type = other RNA
cagggattttcacacatcaa

SEQ ID NO: 22348 - RNA, 20 nt, synthetic construct
  source 1..20: mol_type = other RNA
ggattttcacacatcaaagg

SEQ ID NO: 22349 - RNA, 20 nt, synthetic construct
  source 1..20: mol_type = other RNA
cctctgctctagttgatgtg

SEQ ID NO: 22350 - RNA, 20 nt, synthetic construct
  source 1..20: mol_type = other RNA
cctcacatcaactagagcag

SEQ ID NO: 22351 - RNA, 20 nt, synthetic construct
  source 1..20: mol_type = other RNA
ctctagttgatgtgaggatg

SEQ ID NO: 22352 - RNA, 20 nt, synthetic construct
  source 1..20: mol_type = other RNA
tctagttgatgtgaggatga

SEQ ID NO: 22353 - RNA, 20 nt, synthetic construct
  source 1..20: mol_type = other RNA
ctagttgatgtgaggatgag

SEQ ID NO: 22354 - RNA, 20 nt, synthetic construct
  source 1..20: mol_type = other RNA
tagttgatgtgaggatgagg

SEQ ID NO: 22355 - RNA, 20 nt, synthetic construct
  source 1..20: mol_type = other RNA
ttgatgtgaggatgaggggg

SEQ ID NO: 22356 - RNA, 20 nt, synthetic construct
  source 1..20: mol_type = other RNA
gcctagaccccctgctgccc

SEQ ID NO: 22357 - RNA, 20 nt, synthetic construct
  source 1..20: mol_type = other RNA
gcctgggcagcagggggtct

SEQ ID NO: 22358 - RNA, 20 nt, synthetic construct
  source 1..20: mol_type = other RNA
ccctgctgcccaggccgttg

SEQ ID NO: 22359 - RNA, 20 nt, synthetic construct
  source 1..20: mol_type = other RNA
tcaacggcctgggcagcagg

SEQ ID NO: 22360 - RNA, 20 nt, synthetic construct
  source 1..20: mol_type = other RNA
ctcaacggcctgggcagcag

SEQ ID NO: 22361 - RNA, 20 nt, synthetic construct
  source 1..20: mol_type = other RNA
cctcaacggcctgggcagca

SEQ ID NO: 22362 - RNA, 20 nt, synthetic construct
  source 1..20: mol_type = other RNA
gcctcaacggcctgggcagc

SEQ ID NO: 22363 - RNA, 20 nt, synthetic construct
  source 1..20: mol_type = other RNA
ccaggccgttgaggcaacac

SEQ ID NO: 22364 - RNA, 20 nt, synthetic construct
  source 1..20: mol_type = other RNA
caggccgttgaggcaacact

SEQ ID NO: 22365 - RNA, 20 nt, synthetic construct
  source 1..20: mol_type = other RNA
cagtgttgcctcaacggcct

SEQ ID NO: 22366 - RNA, 20 nt, synthetic construct
  source 1..20: mol_type = other RNA
ccagtgttgcctcaacggcc

SEQ ID NO: 22367 - RNA, 20 nt, synthetic construct
  source 1..20: mol_type = other RNA
ttgaggcaacactgggttcc

SEQ ID NO: 22368 - RNA, 20 nt, synthetic construct
  source 1..20: mol_type = other RNA
ggaacccagtgttgcctcaa

SEQ ID NO: 22369 - RNA, 20 nt, synthetic construct
  source 1..20: mol_type = other RNA
ggttcctggcttgacagctg

SEQ ID NO: 22370 - RNA, 20 nt, synthetic construct
  source 1..20: mol_type = other RNA
gttcctggcttgacagctgt

SEQ ID NO: 22371 - RNA, 20 nt, synthetic construct
  source 1..20: mol_type = other RNA
ctggcttgacagctgtgggc

SEQ ID NO: 22372 - RNA, 20 nt, synthetic construct
  source 1..20: mol_type = other RNA
cagcccacagctgtcaagcc

SEQ ID NO: 22373 - RNA, 20 nt, synthetic construct
  source 1..20: mol_type = other RNA
gctgcccttgccagctcaga

SEQ ID NO: 22374 - RNA, 20 nt, synthetic construct
  source 1..20: mol_type = other RNA
cccttgccagctcagacggc

SEQ ID NO: 22375 - RNA, 20 nt, synthetic construct
  source 1..20: mol_type = other RNA
ccagccgtctgagctggcaa

SEQ ID NO: 22376 - RNA, 20 nt, synthetic construct
  source 1..20: mol_type = other RNA
gccagccgtctgagctggca

SEQ ID NO: 22377 - RNA, 20 nt, synthetic construct
  source 1..20: mol_type = other RNA
aactcgccagccgtctgagc

SEQ ID NO: 22378 - RNA, 20 nt, synthetic construct
  source 1..20: mol_type = other RNA
gcgagttttcagcttcccta

SEQ ID NO: 22379 - RNA, 20 nt, synthetic construct
  source 1..20: mol_type = other RNA
cgagttttcagcttccctaa

SEQ ID NO: 22380 - RNA, 20 nt, synthetic construct
  source 1..20: mol_type = other RNA
tttcagcttccctaagggac

SEQ ID NO: 22381 - RNA, 20 nt, synthetic construct
  source 1..20: mol_type = other RNA
cttccctaagggactggcat

SEQ ID NO: 22382 - RNA, 20 nt, synthetic construct
  source 1..20: mol_type = other RNA
ttccctaagggactggcata

SEQ ID NO: 22383 - RNA, 20 nt, synthetic construct
  source 1..20: mol_type = other RNA
aaccctatgccagtccctta

SEQ ID NO: 22384 - RNA, 20 nt, synthetic construct
  source 1..20: mol_type = other RNA
aaaccctatgccagtccctt

SEQ ID NO: 22385 - RNA, 20 nt, synthetic construct
  source 1..20: mol_type = other RNA
ggactggcatagggttttgt

SEQ ID NO: 22386 - RNA, 20 nt, synthetic construct
  source 1..20: mol_type = other RNA
gactggcatagggttttgtg

SEQ ID NO: 22387 - RNA, 20 nt, synthetic construct
  source 1..20: mol_type = other RNA
ggttttgtggggtcaatgcc

SEQ ID NO: 22388 - RNA, 20 nt, synthetic construct
  source 1..20: mol_type = other RNA
tggggtcaatgccaggaacc

SEQ ID NO: 22389 - RNA, 20 nt, synthetic construct
  source 1..20: mol_type = other RNA
ggggtcaatgccaggaacct

SEQ ID NO: 22390 - RNA, 20 nt, synthetic construct
  source 1..20: mol_type = other RNA
gggtcaatgccaggaacctg

SEQ ID NO: 22391 - RNA, 20 nt, synthetic construct
  source 1..20: mol_type = other RNA
ggtcaatgccaggaacctgg

SEQ ID NO: 22392 - RNA, 20 nt, synthetic construct
  source 1..20: mol_type = other RNA
gccaggaacctgggggaaac

SEQ ID NO: 22393 - RNA, 20 nt, synthetic construct
  source 1..20: mol_type = other RNA
tccagtttcccccaggttcc

SEQ ID NO: 22394 - RNA, 20 nt, synthetic construct
  source 1..20: mol_type = other RNA
aaacgcatccagtttccccc

SEQ ID NO: 22395 - RNA, 20 nt, synthetic construct
  source 1..20: mol_type = other RNA
gcaggagggatgaacttctt

SEQ ID NO: 22396 - RNA, 20 nt, synthetic construct
  source 1..20: mol_type = other RNA
cctcctgctcttactgtttc

SEQ ID NO: 22397 - RNA, 20 nt, synthetic construct
  source 1..20: mol_type = other RNA
cggaaacagtaagagcagga

SEQ ID NO: 22398 - RNA, 20 nt, synthetic construct
  source 1..20: mol_type = other RNA
ccggaaacagtaagagcagg

SEQ ID NO: 22399 - RNA, 20 nt, synthetic construct
  source 1..20: mol_type = other RNA
gctcttactgtttccggccc

SEQ ID NO: 22400 - RNA, 20 nt, synthetic construct
  source 1..20: mol_type = other RNA
gggccggaaacagtaagagc

SEQ ID NO: 22401 - RNA, 20 nt, synthetic construct
  source 1..20: mol_type = other RNA
cttactgtttccggccctgg

SEQ ID NO: 22402 - RNA, 20 nt, synthetic construct
  source 1..20: mol_type = other RNA
tccggccctggaggagaatg

SEQ ID NO: 22403 - RNA, 20 nt, synthetic construct
  source 1..20: mol_type = other RNA
ccggccctggaggagaatga

SEQ ID NO: 22404 - RNA, 20 nt, synthetic construct
  source 1..20: mol_type = other RNA
gccctggaggagaatgaggg

SEQ ID NO: 22405 - RNA, 20 nt, synthetic construct
  source 1..20: mol_type = other RNA
ccctcattctcctccagggc

SEQ ID NO: 22406 - RNA, 20 nt, synthetic construct
  source 1..20: mol_type = other RNA
ggaggagaatgagggaggag

SEQ ID NO: 22407 - RNA, 20 nt, synthetic construct
  source 1..20: mol_type = other RNA
tcctccctcattctcctcca

SEQ ID NO: 22408 - RNA, 20 nt, synthetic construct
  source 1..20: mol_type = other RNA
ctcctccctcattctcctcc

SEQ ID NO: 22409 - RNA, 20 nt, synthetic construct
  source 1..20: mol_type = other RNA
tagcttttattattagcaag

SEQ ID NO: 22410 - RNA, 20 nt, synthetic construct
  source 1..20: mol_type = other RNA
agcttttattattagcaaga

SEQ ID NO: 22411 - RNA, 20 nt, synthetic construct
  source 1..20: mol_type = other RNA
tttcatgcacaaattacaaa

SEQ ID NO: 22412 - RNA, 20 nt, synthetic construct
  source 1..20: mol_type = other RNA
atgaaattcatgtcatttcc

SEQ ID NO: 22413 - RNA, 20 nt, synthetic construct
  source 1..20: mol_type = other RNA
tgaaattcatgtcatttcct

SEQ ID NO: 22414 - RNA, 20 nt, synthetic construct
  source 1..20: mol_type = other RNA
ttcatgtcatttcctgggag

SEQ ID NO: 22415 - RNA, 20 nt, synthetic construct
  source 1..20: mol_type = other RNA
gtcatttcctgggagaggag

SEQ ID NO: 22416 - RNA, 20 nt, synthetic construct
  source 1..20: mol_type = other RNA
tcatttcctgggagaggaga

SEQ ID NO: 22417 - RNA, 20 nt, synthetic construct
  source 1..20: mol_type = other RNA
tgggagaggagagggccgac

SEQ ID NO: 22418 - RNA, 20 nt, synthetic construct
  source 1..20: mol_type = other RNA
agtcggccctctcctctccc

SEQ ID NO: 22419 - RNA, 20 nt, synthetic construct
  source 1..20: mol_type = other RNA
gaggagagggccgactggag

SEQ ID NO: 22420 - RNA, 20 nt, synthetic construct
  source 1..20: mol_type = other RNA
aggagagggccgactggaga

SEQ ID NO: 22421 - RNA, 20 nt, synthetic construct
  source 1..20: mol_type = other RNA
agagggccgactggagaggg

SEQ ID NO: 22422 - RNA, 20 nt, synthetic construct
  source 1..20: mol_type = other RNA
gagggccgactggagagggt

SEQ ID NO: 22423 - RNA, 20 nt, synthetic construct
  source 1..20: mol_type = other RNA
agggccgactggagagggtg

SEQ ID NO: 22424 - RNA, 20 nt, synthetic construct
  source 1..20: mol_type = other RNA
gggccgactggagagggtgg

SEQ ID NO: 22425 - RNA, 20 nt, synthetic construct
  source 1..20: mol_type = other RNA
ggccgactggagagggtggg

SEQ ID NO: 22426 - RNA, 20 nt, synthetic construct
  source 1..20: mol_type = other RNA
tgccccccaccctctccagt

SEQ ID NO: 22427 - RNA, 20 nt, synthetic construct
  source 1..20: mol_type = other RNA
ggagagggtggggggcacac

SEQ ID NO: 22428 - RNA, 20 nt, synthetic construct
  source 1..20: mol_type = other RNA
gagagggtggggggcacact

SEQ ID NO: 22429 - RNA, 20 nt, synthetic construct
  source 1..20: mol_type = other RNA
agagggtggggggcacactg

SEQ ID NO: 22430 - RNA, 20 nt, synthetic construct
  source 1..20: mol_type = other RNA
ggggggcacactggggaagc

SEQ ID NO: 22431 - RNA, 20 nt, synthetic construct
  source 1..20: mol_type = other RNA
cacactggggaagcaggcag

SEQ ID NO: 22432 - RNA, 20 nt, synthetic construct
  source 1..20: mol_type = other RNA
cagaggtttccttcccttgt

SEQ ID NO: 22433 - RNA, 20 nt, synthetic construct
  source 1..20: mol_type = other RNA
agaggtttccttcccttgta

SEQ ID NO: 22434 - RNA, 20 nt, synthetic construct
  source 1..20: mol_type = other RNA
gaggtttccttcccttgtag

SEQ ID NO: 22435 - RNA, 20 nt, synthetic construct
  source 1..20: mol_type = other RNA
aggtttccttcccttgtagg

SEQ ID NO: 22436 - RNA, 20 nt, synthetic construct
  source 1..20: mol_type = other RNA
ggtttccttcccttgtaggg

SEQ ID NO: 22437 - RNA, 20 nt, synthetic construct
  source 1..20: mol_type = other RNA
ttccttcccttgtagggggg

SEQ ID NO: 22438 - RNA, 20 nt, synthetic construct
  source 1..20: mol_type = other RNA
tccttcccttgtaggggggt

SEQ ID NO: 22439 - RNA, 20 nt, synthetic construct
  source 1..20: mol_type = other RNA
ccttcccttgtaggggggtg

SEQ ID NO: 22440 - RNA, 20 nt, synthetic construct
  source 1..20: mol_type = other RNA
ccccacccccctacaaggga

SEQ ID NO: 22441 - RNA, 20 nt, synthetic construct
  source 1..20: mol_type = other RNA
ttgtaggggggtggggagag

SEQ ID NO: 22442 - RNA, 20 nt, synthetic construct
  source 1..20: mol_type = other RNA
tgtaggggggtggggagagt

SEQ ID NO: 22443 - RNA, 20 nt, synthetic construct
  source 1..20: mol_type = other RNA
ctctccccacccccctacaa

SEQ ID NO: 22444 - RNA, 20 nt, synthetic construct
  source 1..20: mol_type = other RNA
actctccccacccccctaca

SEQ ID NO: 22445 - RNA, 20 nt, synthetic construct
  source 1..20: mol_type = other RNA
ggggtggggagagtggggag

SEQ ID NO: 22446 - RNA, 20 nt, synthetic construct
  source 1..20: mol_type = other RNA
gggtggggagagtggggaga

SEQ ID NO: 22447 - RNA, 20 nt, synthetic construct
  source 1..20: mol_type = other RNA
ggtggggagagtggggagag

SEQ ID NO: 22448 - RNA, 20 nt, synthetic construct
  source 1..20: mol_type = other RNA
gtggggagagtggggagagg

SEQ ID NO: 22449 - RNA, 20 nt, synthetic construct
  source 1..20: mol_type = other RNA
gctatccagttcgcctgatg

SEQ ID NO: 22450 - RNA, 20 nt, synthetic construct
  source 1..20: mol_type = other RNA
ctatccagttcgcctgatga

SEQ ID NO: 22451 - RNA, 20 nt, synthetic construct
  source 1..20: mol_type = other RNA
agagccctcatcaggcgaac

SEQ ID NO: 22452 - RNA, 20 nt, synthetic construct
  source 1..20: mol_type = other RNA
ctggttcgagagccctcatc

SEQ ID NO: 22453 - RNA, 20 nt, synthetic construct
  source 1..20: mol_type = other RNA
ggctctcgaaccagccgttt

SEQ ID NO: 22454 - RNA, 20 nt, synthetic construct
  source 1..20: mol_type = other RNA
gctctcgaaccagccgtttt

SEQ ID NO: 22455 - RNA, 20 nt, synthetic construct
  source 1..20: mol_type = other RNA
gccgttttgggttgtgttaa

SEQ ID NO: 22456 - RNA, 20 nt, synthetic construct
  source 1..20: mol_type = other RNA
ttaacacaacccaaaacggc

SEQ ID NO: 22457 - RNA, 20 nt, synthetic construct
  source 1..20: mol_type = other RNA
acctttaacacaacccaaaa

SEQ ID NO: 22458 - RNA, 20 nt, synthetic construct
  source 1..20: mol_type = other RNA
gattgtacattaatggagga

SEQ ID NO: 22459 - RNA, 20 nt, synthetic construct
  source 1..20: mol_type = other RNA
tcgagattgtacattaatgg

SEQ ID NO: 22460 - RNA, 20 nt, synthetic construct
  source 1..20: mol_type = other RNA
agttcgagattgtacattaa

SEQ ID NO: 22461 - RNA, 20 nt, synthetic construct
  source 1..20: mol_type = other RNA
cgaactaactgctaataaag

SEQ ID NO: 22462 - RNA, 20 nt, synthetic construct
  source 1..20: mol_type = other RNA
gaactaactgctaataaagt

SEQ ID NO: 22463 - RNA, 20 nt, synthetic construct
  source 1..20: mol_type = other RNA
aactaactgctaataaagtg

SEQ ID NO: 22464 - RNA, 20 nt, synthetic construct
  source 1..20: mol_type = other RNA
taaaagaaatatttattgtg

SEQ ID NO: 22465 - RNA, 20 nt, synthetic construct
  source 1..20: mol_type = other RNA
agaaattgagaaaacagtgt

SEQ ID NO: 22466 - RNA, 20 nt, synthetic construct
  source 1..20: mol_type = other RNA
taaagcctcccacaatccca

SEQ ID NO: 22467 - RNA, 20 nt, synthetic construct
  source 1..20: mol_type = other RNA
ctggaccttgggattgtggg

SEQ ID NO: 22468 - RNA, 20 nt, synthetic construct
  source 1..20: mol_type = other RNA
tctctggaccttgggattgt

SEQ ID NO: 22469 - RNA, 20 nt, synthetic construct
  source 1..20: mol_type = other RNA
atctctggaccttgggattg

SEQ ID NO: 22470 - RNA, 20 nt, synthetic construct
  source 1..20: mol_type = other RNA
ctgtattatctctggacctt

SEQ ID NO: 22471 - RNA, 20 nt, synthetic construct
  source 1..20: mol_type = other RNA
gctgtattatctctggacct

SEQ ID NO: 22472 - RNA, 20 nt, synthetic construct
  source 1..20: mol_type = other RNA
agataatacagctcaagaat

SEQ ID NO: 22473 - RNA, 20 nt, synthetic construct
  source 1..20: mol_type = other RNA
ttcttgagctgtattatctc

SEQ ID NO: 22474 - RNA, 20 nt, synthetic construct
  source 1..20: mol_type = other RNA
acagagaaaaaaaaggaaga

SEQ ID NO: 22475 - RNA, 20 nt, synthetic construct
  source 1..20: mol_type = other RNA
tggagagacagagaaaaaaa

SEQ ID NO: 22476 - RNA, 20 nt, synthetic construct
  source 1..20: mol_type = other RNA
tgtacacatacagatgcaga

SEQ ID NO: 22477 - RNA, 20 nt, synthetic construct
  source 1..20: mol_type = other RNA
gaagagcaagaagagaaaac

SEQ ID NO: 22478 - RNA, 20 nt, synthetic construct
  source 1..20: mol_type = other RNA
tgctcttcacccacaaaagc

SEQ ID NO: 22479 - RNA, 20 nt, synthetic construct
  source 1..20: mol_type = other RNA
ggctggatgcctgcttttgt

SEQ ID NO: 22480 - RNA, 20 nt, synthetic construct
  source 1..20: mol_type = other RNA
aggctggatgcctgcttttg

SEQ ID NO: 22481 - RNA, 20 nt, synthetic construct
  source 1..20: mol_type = other RNA
atgcgagatgctcaaaaggc

SEQ ID NO: 22482 - RNA, 20 nt, synthetic construct
  source 1..20: mol_type = other RNA
tcatatgcgagatgctcaaa

SEQ ID NO: 22483 - RNA, 20 nt, synthetic construct
  source 1..20: mol_type = other RNA
taggtgaggcaggtctttga

SEQ ID NO: 22484 - RNA, 20 nt, synthetic construct
  source 1..20: mol_type = other RNA
gaaatgggcttaggtgaggc

SEQ ID NO: 22485 - RNA, 20 nt, synthetic construct
  source 1..20: mol_type = other RNA
ctgagaaatgggcttaggtg

SEQ ID NO: 22486 - RNA, 20 nt, synthetic construct
  source 1..20: mol_type = other RNA
tgggtctgagaaatgggctt

SEQ ID NO: 22487 - RNA, 20 nt, synthetic construct
  source 1..20: mol_type = other RNA
ccatttctcagacccacctg

SEQ ID NO: 22488 - RNA, 20 nt, synthetic construct
  source 1..20: mol_type = other RNA
cgcaggtgggtctgagaaat

SEQ ID NO: 22489 - RNA, 20 nt, synthetic construct
  source 1..20: mol_type = other RNA
ccgcaggtgggtctgagaaa

SEQ ID NO: 22490 - RNA, 20 nt, synthetic construct
  source 1..20: mol_type = other RNA
gacccacctgcggtctactc

SEQ ID NO: 22491 - RNA, 20 nt, synthetic construct
  source 1..20: mol_type = other RNA
ggcctgagtagaccgcaggt

SEQ ID NO: 22492 - RNA, 20 nt, synthetic construct
  source 1..20: mol_type = other RNA
aggcctgagtagaccgcagg

SEQ ID NO: 22493 - RNA, 20 nt, synthetic construct
  source 1..20: mol_type = other RNA
aggaggcctgagtagaccgc

SEQ ID NO: 22494 - RNA, 20 nt, synthetic construct
  source 1..20: mol_type = other RNA
gggcttggtggatgacaagg

SEQ ID NO: 22495 - RNA, 20 nt, synthetic construct
  source 1..20: mol_type = other RNA
gtcatccaccaagccctctc

SEQ ID NO: 22496 - RNA, 20 nt, synthetic construct
  source 1..20: mol_type = other RNA
agagggcttggtggatgaca

SEQ ID NO: 22497 - RNA, 20 nt, synthetic construct
  source 1..20: mol_type = other RNA
caagccctctctggcttcat

SEQ ID NO: 22498 - RNA, 20 nt, synthetic construct
  source 1..20: mol_type = other RNA
tgaagccagagagggcttgg

SEQ ID NO: 22499 - RNA, 20 nt, synthetic construct
  source 1..20: mol_type = other RNA
caatgaagccagagagggct

SEQ ID NO: 22500 - RNA, 20 nt, synthetic construct
  source 1..20: mol_type = other RNA
agtaccaatgaagccagaga

SEQ ID NO: 22501 - RNA, 20 nt, synthetic construct
  source 1..20: mol_type = other RNA
cagtaccaatgaagccagag

SEQ ID NO: 22502 - RNA, 20 nt, synthetic construct
  source 1..20: mol_type = other RNA
ggcttcattggtactgccgc

SEQ ID NO: 22503 - RNA, 20 nt, synthetic construct
  source 1..20: mol_type = other RNA
ttggtactgccgcaggctgc

SEQ ID NO: 22504 - RNA, 20 nt, synthetic construct
  source 1..20: mol_type = other RNA
tggtactgccgcaggctgct

SEQ ID NO: 22505 - RNA, 20 nt, synthetic construct
  source 1..20: mol_type = other RNA
tactagtgcccagcagcctg

SEQ ID NO: 22506 - RNA, 20 nt, synthetic construct
  source 1..20: mol_type = other RNA
tgctgggcactagtatctcc

SEQ ID NO: 22507 - RNA, 20 nt, synthetic construct
  source 1..20: mol_type = other RNA
tggcgtctctgttgcacctg

SEQ ID NO: 22508 - RNA, 20 nt, synthetic construct
  source 1..20: mol_type = other RNA
tcaggtgcaacagagacgcc

SEQ ID NO: 22509 - RNA, 20 nt, synthetic construct
  source 1..20: mol_type = other RNA
ctgttgcacctgaggttcca

SEQ ID NO: 22510 - RNA, 20 nt, synthetic construct
  source 1..20: mol_type = other RNA
tgcacctgaggttccacggc

SEQ ID NO: 22511 - RNA, 20 nt, synthetic construct
  source 1..20: mol_type = other RNA
cctgaggttccacggctggc

SEQ ID NO: 22512 - RNA, 20 nt, synthetic construct
  source 1..20: mol_type = other RNA
ccagccagccgtggaacctc

SEQ ID NO: 22513 - RNA, 20 nt, synthetic construct
  source 1..20: mol_type = other RNA
ggctggctggtgttccttcc

SEQ ID NO: 22514 - RNA, 20 nt, synthetic construct
  source 1..20: mol_type = other RNA
gaaggaacaccagccagccg

SEQ ID NO: 22515 - RNA, 20 nt, synthetic construct
  source 1..20: mol_type = other RNA
gctggtgttccttcctggaa

SEQ ID NO: 22516 - RNA, 20 nt, synthetic construct
  source 1..20: mol_type = other RNA
ggtgttccttcctggaatgg

SEQ ID NO: 22517 - RNA, 20 nt, synthetic construct
  source 1..20: mol_type = other RNA
gtgttccttcctggaatgga

SEQ ID NO: 22518 - RNA, 20 nt, synthetic construct
  source 1..20: mol_type = other RNA
gttctccctccattccagga

SEQ ID NO: 22519 - RNA, 20 nt, synthetic construct
  source 1..20: mol_type = other RNA
gattgttctccctccattcc

SEQ ID NO: 22520 - RNA, 20 nt, synthetic construct
  source 1..20: mol_type = other RNA
atggagggagaacaatcact

SEQ ID NO: 22521 - RNA, 20 nt, synthetic construct
  source 1..20: mol_type = other RNA
ttatttgagtcccagtagat

SEQ ID NO: 22522 - RNA, 20 nt, synthetic construct
  source 1..20: mol_type = other RNA
tgagtcccagtagattggag

SEQ ID NO: 22523 - RNA, 20 nt, synthetic construct
  source 1..20: mol_type = other RNA
agtagattggagaggtccac

SEQ ID NO: 22524 - RNA, 20 nt, synthetic construct
  source 1..20: mol_type = other RNA
gtggacctctccaatctact

SEQ ID NO: 22525 - RNA, 20 nt, synthetic construct
  source 1..20: mol_type = other RNA
agtggacctctccaatctac

SEQ ID NO: 22526 - RNA, 20 nt, synthetic construct
  source 1..20: mol_type = other RNA
gattggagaggtccactggc

SEQ ID NO: 22527 - RNA, 20 nt, synthetic construct
  source 1..20: mol_type = other RNA
caactaacaaagccggccag

SEQ ID NO: 22528 - RNA, 20 nt, synthetic construct
  source 1..20: mol_type = other RNA
tttgctgcaactaacaaagc

SEQ ID NO: 22529 - RNA, 20 nt, synthetic construct
  source 1..20: mol_type = other RNA
tctctgatggcagtttgagt

SEQ ID NO: 22530 - RNA, 20 nt, synthetic construct
  source 1..20: mol_type = other RNA
agtcgggactgctgtgccta

SEQ ID NO: 22531 - RNA, 20 nt, synthetic construct
  source 1..20: mol_type = other RNA
ataggcacagcagtcccgac

SEQ ID NO: 22532 - RNA, 20 nt, synthetic construct
  source 1..20: mol_type = other RNA
gactgctgtgcctatggagt

SEQ ID NO: 22533 - RNA, 20 nt, synthetic construct
  source 1..20: mol_type = other RNA
taagaagttacctactccat

SEQ ID NO: 22534 - RNA, 20 nt, synthetic construct
  source 1..20: mol_type = other RNA
aaaagaaaaaatgaaaataa

SEQ ID NO: 22535 - RNA, 20 nt, synthetic construct
  source 1..20: mol_type = other RNA
gtaaaaaatttttaatttat

SEQ ID NO: 22536 - RNA, 20 nt, synthetic construct
  source 1..20: mol_type = other RNA
taaaaaatttttaatttata

SEQ ID NO: 22537 - RNA, 20 nt, synthetic construct
  source 1..20: mol_type = other RNA
aaaaaatttttaatttatag

SEQ ID NO: 22538 - RNA, 20 nt, synthetic construct
  source 1..20: mol_type = other RNA
tttaatttataggggttttc

SEQ ID NO: 22539 - RNA, 20 nt, synthetic construct
  source 1..20: mol_type = other RNA
aggggttttctggtaaaaac

SEQ ID NO: 22540 - RNA, 20 nt, synthetic construct
  source 1..20: mol_type = other RNA
tcttttagaatttgtctagc

SEQ ID NO: 22541 - RNA, 20 nt, synthetic construct
  source 1..20: mol_type = other RNA
gaagtttattcagaaaataa

SEQ ID NO: 22542 - RNA, 20 nt, synthetic construct
  source 1..20: mol_type = other RNA
ttccttccactttactctgt

SEQ ID NO: 22543 - RNA, 20 nt, synthetic construct
  source 1..20: mol_type = other RNA
agccaacagagtaaagtgga

SEQ ID NO: 22544 - RNA, 20 nt, synthetic construct
  source 1..20: mol_type = other RNA
agcaagccaacagagtaaag

SEQ ID NO: 22545 - RNA, 20 nt, synthetic construct
  source 1..20: mol_type = other RNA
tacaaagccaagaatccacg

SEQ ID NO: 22546 - RNA, 20 nt, synthetic construct
  source 1..20: mol_type = other RNA
gtggattcttggctttgtac

SEQ ID NO: 22547 - RNA, 20 nt, synthetic construct
  source 1..20: mol_type = other RNA
tgggaggccacgtggattct

SEQ ID NO: 22548 - RNA, 20 nt, synthetic construct
  source 1..20: mol_type = other RNA
gttcagcgtgggaggccacg

SEQ ID NO: 22549 - RNA, 20 nt, synthetic construct
  source 1..20: mol_type = other RNA
cccacgctgaaccccaattt

SEQ ID NO: 22550 - RNA, 20 nt, synthetic construct
  source 1..20: mol_type = other RNA
ccacgctgaaccccaatttt

SEQ ID NO: 22551 - RNA, 20 nt, synthetic construct
  source 1..20: mol_type = other RNA
aaattggggttcagcgtggg

SEQ ID NO: 22552 - RNA, 20 nt, synthetic construct
  source 1..20: mol_type = other RNA
ccaaaattggggttcagcgt

SEQ ID NO: 22553 - RNA, 20 nt, synthetic construct
  source 1..20: mol_type = other RNA
cccaaaattggggttcagcg

SEQ ID NO: 22554 - RNA, 20 nt, synthetic construct
  source 1..20: mol_type = other RNA
cagggtgagccccaaaattg

SEQ ID NO: 22555 - RNA, 20 nt, synthetic construct
  source 1..20: mol_type = other RNA
acagggtgagccccaaaatt

SEQ ID NO: 22556 - RNA, 20 nt, synthetic construct
  source 1..20: mol_type = other RNA
cacagggtgagccccaaaat

SEQ ID NO: 22557 - RNA, 20 nt, synthetic construct
  source 1..20: mol_type = other RNA
tcaccctgtgacacagccag

SEQ ID NO: 22558 - RNA, 20 nt, synthetic construct
  source 1..20: mol_type = other RNA
gtgacacagccagaggcaaa

SEQ ID NO: 22559 - RNA, 20 nt, synthetic construct
  source 1..20: mol_type = other RNA
ttgcctctggctgtgtcaca

SEQ ID NO: 22560 - RNA, 20 nt, synthetic construct
  source 1..20: mol_type = other RNA
tttgcctctggctgtgtcac

SEQ ID NO: 22561 - RNA, 20 nt, synthetic construct
  source 1..20: mol_type = other RNA
gacatggaaccatttgcctc

SEQ ID NO: 22562 - RNA, 20 nt, synthetic construct
  source 1..20: mol_type = other RNA
aaagaggaataggagggaca

SEQ ID NO: 22563 - RNA, 20 nt, synthetic construct
  source 1..20: mol_type = other RNA
ctcctattcctctttgcgcc

SEQ ID NO: 22564 - RNA, 20 nt, synthetic construct
  source 1..20: mol_type = other RNA
aggcgcaaagaggaatagga

SEQ ID NO: 22565 - RNA, 20 nt, synthetic construct
  source 1..20: mol_type = other RNA
tattcctctttgcgcctgga

SEQ ID NO: 22566 - RNA, 20 nt, synthetic construct
  source 1..20: mol_type = other RNA
attcctctttgcgcctggat

SEQ ID NO: 22567 - RNA, 20 nt, synthetic construct
  source 1..20: mol_type = other RNA
atccaggcgcaaagaggaat

SEQ ID NO: 22568 - RNA, 20 nt, synthetic construct
  source 1..20: mol_type = other RNA
ctttgcgcctggatgggatc

SEQ ID NO: 22569 - RNA, 20 nt, synthetic construct
  source 1..20: mol_type = other RNA
gatcccatccaggcgcaaag

SEQ ID NO: 22570 - RNA, 20 nt, synthetic construct
  source 1..20: mol_type = other RNA
tgcgcctggatgggatccgg

SEQ ID NO: 22571 - RNA, 20 nt, synthetic construct
  source 1..20: mol_type = other RNA
gcgcctggatgggatccgga

SEQ ID NO: 22572 - RNA, 20 nt, synthetic construct
  source 1..20: mol_type = other RNA
gatgggatccggagggctct

SEQ ID NO: 22573 - RNA, 20 nt, synthetic construct
  source 1..20: mol_type = other RNA
gagccctccggatcccatcc

SEQ ID NO: 22574 - RNA, 20 nt, synthetic construct
  source 1..20: mol_type = other RNA
gatccggagggctctaggct

SEQ ID NO: 22575 - RNA, 20 nt, synthetic construct
  source 1..20: mol_type = other RNA
cagccaagcctagagccctc

SEQ ID NO: 22576 - RNA, 20 nt, synthetic construct
  source 1..20: mol_type = other RNA
ggctctaggcttggctgctg

SEQ ID NO: 22577 - RNA, 20 nt, synthetic construct
  source 1..20: mol_type = other RNA
gctgctgtggccaccagatg

SEQ ID NO: 22578 - RNA, 20 nt, synthetic construct
  source 1..20: mol_type = other RNA
ccaccagatgaggctctatg

SEQ ID NO: 22579 - RNA, 20 nt, synthetic construct
  source 1..20: mol_type = other RNA
cctcatagagcctcatctgg

SEQ ID NO: 22580 - RNA, 20 nt, synthetic construct
  source 1..20: mol_type = other RNA
tgaggctctatgaggtctgc

SEQ ID NO: 22581 - RNA, 20 nt, synthetic construct
  source 1..20: mol_type = other RNA
gaggctctatgaggtctgca

SEQ ID NO: 22582 - RNA, 20 nt, synthetic construct
  source 1..20: mol_type = other RNA
aggctctatgaggtctgcag

SEQ ID NO: 22583 - RNA, 20 nt, synthetic construct
  source 1..20: mol_type = other RNA
ggggtcttgccagctccaga

SEQ ID NO: 22584 - RNA, 20 nt, synthetic construct
  source 1..20: mol_type = other RNA
agggaatgtccatctggagc

SEQ ID NO: 22585 - RNA, 20 nt, synthetic construct
  source 1..20: mol_type = other RNA
catctcagggaatgtccatc

SEQ ID NO: 22586 - RNA, 20 nt, synthetic construct
  source 1..20: mol_type = other RNA
acattccctgagatgctgtt

SEQ ID NO: 22587 - RNA, 20 nt, synthetic construct
  source 1..20: mol_type = other RNA
tgagatgctgttaggccacc

SEQ ID NO: 22588 - RNA, 20 nt, synthetic construct
  source 1..20: mol_type = other RNA
ggtggcctaacagcatctca

SEQ ID NO: 22589 - RNA, 20 nt, synthetic construct
  source 1..20: mol_type = other RNA
aggtggcctaacagcatctc

SEQ ID NO: 22590 - RNA, 20 nt, synthetic construct
  source 1..20: mol_type = other RNA
tgctgttaggccacctggac

SEQ ID NO: 22591 - RNA, 20 nt, synthetic construct
  source 1..20: mol_type = other RNA
gctgttaggccacctggact

SEQ ID NO: 22592 - RNA, 20 nt, synthetic construct
  source 1..20: mol_type = other RNA
ctgttaggccacctggactg

SEQ ID NO: 22593 - RNA, 20 nt, synthetic construct
  source 1..20: mol_type = other RNA
acctggactggggccccctg

SEQ ID NO: 22594 - RNA, 20 nt, synthetic construct
  source 1..20: mol_type = other RNA
acagggggccccagtccagg

SEQ ID NO: 22595 - RNA, 20 nt, synthetic construct
  source 1..20: mol_type = other RNA
gccacagggggccccagtcc

SEQ ID NO: 22596 - RNA, 20 nt, synthetic construct
  source 1..20: mol_type = other RNA
ggggccccctgtggcatccc

SEQ ID NO: 22597 - RNA, 20 nt, synthetic construct
  source 1..20: mol_type = other RNA
cccctgtggcatccctggca

SEQ ID NO: 22598 - RNA, 20 nt, synthetic construct
  source 1..20: mol_type = other RNA
catgccagggatgccacagg

SEQ ID NO: 22599 - RNA, 20 nt, synthetic construct
  source 1..20: mol_type = other RNA
ccatgccagggatgccacag

SEQ ID NO: 22600 - RNA, 20 nt, synthetic construct
  source 1..20: mol_type = other RNA
tccatgccagggatgccaca

SEQ ID NO: 22601 - RNA, 20 nt, synthetic construct
  source 1..20: mol_type = other RNA
gtccatgccagggatgccac

SEQ ID NO: 22602 - RNA, 20 nt, synthetic construct
  source 1..20: mol_type = other RNA
ggcattatgtgtccatgcca

SEQ ID NO: 22603 - RNA, 20 nt, synthetic construct
  source 1..20: mol_type = other RNA
gggcattatgtgtccatgcc

SEQ ID NO: 22604 - RNA, 20 nt, synthetic construct
  source 1..20: mol_type = other RNA
ggacacataatgcccagcaa

SEQ ID NO: 22605 - RNA, 20 nt, synthetic construct
  source 1..20: mol_type = other RNA
actttgatgatgcctttgct

SEQ ID NO: 22606 - RNA, 20 nt, synthetic construct
  source 1..20: mol_type = other RNA
aactttgatgatgcctttgc

SEQ ID NO: 22607 - RNA, 20 nt, synthetic construct
  source 1..20: mol_type = other RNA
aagttccattactttagtgc

SEQ ID NO: 22608 - RNA, 20 nt, synthetic construct
  source 1..20: mol_type = other RNA
tccattactttagtgctgga

SEQ ID NO: 22609 - RNA, 20 nt, synthetic construct
  source 1..20: mol_type = other RNA
gccttccagcactaaagtaa

SEQ ID NO: 22610 - RNA, 20 nt, synthetic construct
  source 1..20: mol_type = other RNA
gtgctggaaggcaaaccaga

SEQ ID NO: 22611 - RNA, 20 nt, synthetic construct
  source 1..20: mol_type = other RNA
tctgcaaacaagttgccatc

SEQ ID NO: 22612 - RNA, 20 nt, synthetic construct
  source 1..20: mol_type = other RNA
aagaaactgagacccaaaga

SEQ ID NO: 22613 - RNA, 20 nt, synthetic construct
  source 1..20: mol_type = other RNA
agaaactgagacccaaagaa

SEQ ID NO: 22614 - RNA, 20 nt, synthetic construct
  source 1..20: mol_type = other RNA
aagaagggtcagccaaagcc

SEQ ID NO: 22615 - RNA, 20 nt, synthetic construct
  source 1..20: mol_type = other RNA
gctttggctgacccttcttt

SEQ ID NO: 22616 - RNA, 20 nt, synthetic construct
  source 1..20: mol_type = other RNA
ggctttggctgacccttctt

SEQ ID NO: 22617 - RNA, 20 nt, synthetic construct
  source 1..20: mol_type = other RNA
tcagccaaagccaggactca

SEQ ID NO: 22618 - RNA, 20 nt, synthetic construct
  source 1..20: mol_type = other RNA
cagccaaagccaggactcaa

SEQ ID NO: 22619 - RNA, 20 nt, synthetic construct
  source 1..20: mol_type = other RNA
aagccaggactcaagggtca

SEQ ID NO: 22620 - RNA, 20 nt, synthetic construct
  source 1..20: mol_type = other RNA
agccaggactcaagggtcaa

SEQ ID NO: 22621 - RNA, 20 nt, synthetic construct
  source 1..20: mol_type = other RNA
tgacccttgagtcctggctt

SEQ ID NO: 22622 - RNA, 20 nt, synthetic construct
  source 1..20: mol_type = other RNA
aggactcaagggtcaagggc

SEQ ID NO: 22623 - RNA, 20 nt, synthetic construct
  source 1..20: mol_type = other RNA
agcccttgacccttgagtcc

SEQ ID NO: 22624 - RNA, 20 nt, synthetic construct
  source 1..20: mol_type = other RNA
ttgatacttcagctgctgag

SEQ ID NO: 22625 - RNA, 20 nt, synthetic construct
  source 1..20: mol_type = other RNA
tacttcagctgctgagtggc

SEQ ID NO: 22626 - RNA, 20 nt, synthetic construct
  source 1..20: mol_type = other RNA
tgggagaagggcagcaaaaa

SEQ ID NO: 22627 - RNA, 20 nt, synthetic construct
  source 1..20: mol_type = other RNA
ctgggagaagggcagcaaaa

SEQ ID NO: 22628 - RNA, 20 nt, synthetic construct
  source 1..20: mol_type = other RNA
tctcccagagttccataatg

SEQ ID NO: 22629 - RNA, 20 nt, synthetic construct
  source 1..20: mol_type = other RNA
attatggaactctgggagaa

SEQ ID NO: 22630 - RNA, 20 nt, synthetic construct
  source 1..20: mol_type = other RNA
cattatggaactctgggaga

SEQ ID NO: 22631 - RNA, 20 nt, synthetic construct
  source 1..20: mol_type = other RNA
cagagttccataatgaggtg

SEQ ID NO: 22632 - RNA, 20 nt, synthetic construct
  source 1..20: mol_type = other RNA
tcacctcattatggaactct

SEQ ID NO: 22633 - RNA, 20 nt, synthetic construct
  source 1..20: mol_type = other RNA
gttccataatgaggtgagga

SEQ ID NO: 22634 - RNA, 20 nt, synthetic construct
  source 1..20: mol_type = other RNA
ttccataatgaggtgaggat

SEQ ID NO: 22635 - RNA, 20 nt, synthetic construct
  source 1..20: mol_type = other RNA
gacccatcctcacctcatta

SEQ ID NO: 22636 - RNA, 20 nt, synthetic construct
  source 1..20: mol_type = other RNA
ggtgaggatgggtctccttc

SEQ ID NO: 22637 - RNA, 20 nt, synthetic construct
  source 1..20: mol_type = other RNA
gtgaggatgggtctccttca

SEQ ID NO: 22638 - RNA, 20 nt, synthetic construct
  source 1..20: mol_type = other RNA
gatgggtctccttcagggct

SEQ ID NO: 22639 - RNA, 20 nt, synthetic construct
  source 1..20: mol_type = other RNA
tggactctaccaagccctga

SEQ ID NO: 22640 - RNA, 20 nt, synthetic construct
  source 1..20: mol_type = other RNA
agagtccatctttgcacttc

SEQ ID NO: 22641 - RNA, 20 nt, synthetic construct
  source 1..20: mol_type = other RNA
atctttgcacttccggtccc

SEQ ID NO: 22642 - RNA, 20 nt, synthetic construct
  source 1..20: mol_type = other RNA
tgggaccggaagtgcaaaga

SEQ ID NO: 22643 - RNA, 20 nt, synthetic construct
  source 1..20: mol_type = other RNA
tgcacttccggtcccaggac

SEQ ID NO: 22644 - RNA, 20 nt, synthetic construct
  source 1..20: mol_type = other RNA
gcttgagccagtcctgggac

SEQ ID NO: 22645 - RNA, 20 nt, synthetic construct
  source 1..20: mol_type = other RNA
gttcagcttgagccagtcct

SEQ ID NO: 22646 - RNA, 20 nt, synthetic construct
  source 1..20: mol_type = other RNA
tgttcagcttgagccagtcc

SEQ ID NO: 22647 - RNA, 20 nt, synthetic construct
  source 1..20: mol_type = other RNA
agctgaacagcttccgcatc

SEQ ID NO: 22648 - RNA, 20 nt, synthetic construct
  source 1..20: mol_type = other RNA
gaacagcttccgcatctggc

SEQ ID NO: 22649 - RNA, 20 nt, synthetic construct
  source 1..20: mol_type = other RNA
aacagcttccgcatctggct

SEQ ID NO: 22650 - RNA, 20 nt, synthetic construct
  source 1..20: mol_type = other RNA
acacgaggcccagccagatg

SEQ ID NO: 22651 - RNA, 20 nt, synthetic construct
  source 1..20: mol_type = other RNA
gggtgctggctgagaacacg

SEQ ID NO: 22652 - RNA, 20 nt, synthetic construct
  source 1..20: mol_type = other RNA
gcaccctctcgtactgctcc

SEQ ID NO: 22653 - RNA, 20 nt, synthetic construct
  source 1..20: mol_type = other RNA
ggagcagtacgagagggtgc

SEQ ID NO: 22654 - RNA, 20 nt, synthetic construct
  source 1..20: mol_type = other RNA
gagccaggagcagtacgaga

SEQ ID NO: 22655 - RNA, 20 nt, synthetic construct
  source 1..20: mol_type = other RNA
tgagccaggagcagtacgag

SEQ ID NO: 22656 - RNA, 20 nt, synthetic construct
  source 1..20: mol_type = other RNA
gcatggacaggtgctgagcc

SEQ ID NO: 22657 - RNA, 20 nt, synthetic construct
  source 1..20: mol_type = other RNA
cttggacaaactgcatggac

SEQ ID NO: 22658 - RNA, 20 nt, synthetic construct
  source 1..20: mol_type = other RNA
gttgtcttggacaaactgca

SEQ ID NO: 22659 - RNA, 20 nt, synthetic construct
  source 1..20: mol_type = other RNA
gacatcggtggaggttgtct

SEQ ID NO: 22660 - RNA, 20 nt, synthetic construct
  source 1..20: mol_type = other RNA
caacctccaccgatgtcact

SEQ ID NO: 22661 - RNA, 20 nt, synthetic construct
  source 1..20: mol_type = other RNA
aacctccaccgatgtcactc

SEQ ID NO: 22662 - RNA, 20 nt, synthetic construct
  source 1..20: mol_type = other RNA
agcccgagtgacatcggtgg

SEQ ID NO: 22663 - RNA, 20 nt, synthetic construct
  source 1..20: mol_type = other RNA
gatagcccgagtgacatcgg

SEQ ID NO: 22664 - RNA, 20 nt, synthetic construct
  source 1..20: mol_type = other RNA
gctgatagcccgagtgacat

SEQ ID NO: 22665 - RNA, 20 nt, synthetic construct
  source 1..20: mol_type = other RNA
ctatcagctgctctcgatac

SEQ ID NO: 22666 - RNA, 20 nt, synthetic construct
  source 1..20: mol_type = other RNA
tccacaaagtgcagcaactg

SEQ ID NO: 22667 - RNA, 20 nt, synthetic construct
  source 1..20: mol_type = other RNA
ccacaaagtgcagcaactgc

SEQ ID NO: 22668 - RNA, 20 nt, synthetic construct
  source 1..20: mol_type = other RNA
cacaaagtgcagcaactgcg

SEQ ID NO: 22669 - RNA, 20 nt, synthetic construct
  source 1..20: mol_type = other RNA
cccgcagttgctgcactttg

SEQ ID NO: 22670 - RNA, 20 nt, synthetic construct
  source 1..20: mol_type = other RNA
agcaactgcggggcatccag

SEQ ID NO: 22671 - RNA, 20 nt, synthetic construct
  source 1..20: mol_type = other RNA
tgcggggcatccagaggtga

SEQ ID NO: 22672 - RNA, 20 nt, synthetic construct
  source 1..20: mol_type = other RNA
ggcatccagaggtgaaggta

SEQ ID NO: 22673 - RNA, 20 nt, synthetic construct
  source 1..20: mol_type = other RNA
tccagaggtgaaggtacggc

SEQ ID NO: 22674 - RNA, 20 nt, synthetic construct
  source 1..20: mol_type = other RNA
gccagccgtaccttcacctc

SEQ ID NO: 22675 - RNA, 20 nt, synthetic construct
  source 1..20: mol_type = other RNA
cggctggcaacgaacaaaga

SEQ ID NO: 22676 - RNA, 20 nt, synthetic construct
  source 1..20: mol_type = other RNA
ggctggcaacgaacaaagaa

SEQ ID NO: 22677 - RNA, 20 nt, synthetic construct
  source 1..20: mol_type = other RNA
ttggaggtggaggctgtggt

SEQ ID NO: 22678 - RNA, 20 nt, synthetic construct
  source 1..20: mol_type = other RNA
gggattggaggtggaggctg

SEQ ID NO: 22679 - RNA, 20 nt, synthetic construct
  source 1..20: mol_type = other RNA
aaggtggggattggaggtgg

SEQ ID NO: 22680 - RNA, 20 nt, synthetic construct
  source 1..20: mol_type = other RNA
ctgaaggtggggattggagg

SEQ ID NO: 22681 - RNA, 20 nt, synthetic construct
  source 1..20: mol_type = other RNA
gcactgaaggtggggattgg

SEQ ID NO: 22682 - RNA, 20 nt, synthetic construct
  source 1..20: mol_type = other RNA
aaagcactgaaggtggggat

SEQ ID NO: 22683 - RNA, 20 nt, synthetic construct
  source 1..20: mol_type = other RNA
agaggaaagcactgaaggtg

SEQ ID NO: 22684 - RNA, 20 nt, synthetic construct
  source 1..20: mol_type = other RNA
gagaggaaagcactgaaggt

SEQ ID NO: 22685 - RNA, 20 nt, synthetic construct
  source 1..20: mol_type = other RNA
agagaggaaagcactgaagg

SEQ ID NO: 22686 - RNA, 20 nt, synthetic construct
  source 1..20: mol_type = other RNA
atgagagaggaaagcactga

SEQ ID NO: 22687 - RNA, 20 nt, synthetic construct
  source 1..20: mol_type = other RNA
gagggatgcagagatgagag

SEQ ID NO: 22688 - RNA, 20 nt, synthetic construct
  source 1..20: mol_type = other RNA
ctggaggcagaaggaagcga

SEQ ID NO: 22689 - RNA, 20 nt, synthetic construct
  source 1..20: mol_type = other RNA
tctggaggcagaaggaagcg

SEQ ID NO: 22690 - RNA, 20 nt, synthetic construct
  source 1..20: mol_type = other RNA
ggtgcatttctggaggcaga

SEQ ID NO: 22691 - RNA, 20 nt, synthetic construct
  source 1..20: mol_type = other RNA
ggacacaggtgcatttctgg

SEQ ID NO: 22692 - RNA, 20 nt, synthetic construct
  source 1..20: mol_type = other RNA
cctcacaaagagtcaggccc

SEQ ID NO: 22693 - RNA, 20 nt, synthetic construct
  source 1..20: mol_type = other RNA
tgcaaacctcacaaagagtc

SEQ ID NO: 22694 - RNA, 20 nt, synthetic construct
  source 1..20: mol_type = other RNA
gaagggaagagagaaaggaa

SEQ ID NO: 22695 - RNA, 20 nt, synthetic construct
  source 1..20: mol_type = other RNA
ggaagggaagagagaaagga

SEQ ID NO: 22696 - RNA, 20 nt, synthetic construct
  source 1..20: mol_type = other RNA
tgggggaagggaagagagaa

SEQ ID NO: 22697 - RNA, 20 nt, synthetic construct
  source 1..20: mol_type = other RNA
actgtctggttctgggggaa

SEQ ID NO: 22698 - RNA, 20 nt, synthetic construct
  source 1..20: mol_type = other RNA
tactgtctggttctggggga

SEQ ID NO: 22699 - RNA, 20 nt, synthetic construct
  source 1..20: mol_type = other RNA
ggggtactgtctggttctgg

SEQ ID NO: 22700 - RNA, 20 nt, synthetic construct
  source 1..20: mol_type = other RNA
tggggtactgtctggttctg

SEQ ID NO: 22701 - RNA, 20 nt, synthetic construct
  source 1..20: mol_type = other RNA
ctggggtactgtctggttct

SEQ ID NO: 22702 - RNA, 20 nt, synthetic construct
  source 1..20: mol_type = other RNA
tctggggtactgtctggttc

SEQ ID NO: 22703 - RNA, 20 nt, synthetic construct
  source 1..20: mol_type = other RNA
ggcagttctggggtactgtc

SEQ ID NO: 22704 - RNA, 20 nt, synthetic construct
  source 1..20: mol_type = other RNA
agaactgccaccgcctcctg

SEQ ID NO: 22705 - RNA, 20 nt, synthetic construct
  source 1..20: mol_type = other RNA
aggaggcggtggcagttctg

SEQ ID NO: 22706 - RNA, 20 nt, synthetic construct
  source 1..20: mol_type = other RNA
caggaggcggtggcagttct

SEQ ID NO: 22707 - RNA, 20 nt, synthetic construct
  source 1..20: mol_type = other RNA
acaggaggcggtggcagttc

SEQ ID NO: 22708 - RNA, 20 nt, synthetic construct
  source 1..20: mol_type = other RNA
tcagagaccacaggaggcgg

SEQ ID NO: 22709 - RNA, 20 nt, synthetic construct
  source 1..20: mol_type = other RNA
ctctcagagaccacaggagg

SEQ ID NO: 22710 - RNA, 20 nt, synthetic construct
  source 1..20: mol_type = other RNA
cagctctcagagaccacagg

SEQ ID NO: 22711 - RNA, 20 nt, synthetic construct
  source 1..20: mol_type = other RNA
taacagctctcagagaccac

SEQ ID NO: 22712 - RNA, 20 nt, synthetic construct
  source 1..20: mol_type = other RNA
agagctgttactgacctatg

SEQ ID NO: 22713 - RNA, 20 nt, synthetic construct
  source 1..20: mol_type = other RNA
gagctgttactgacctatgc

SEQ ID NO: 22714 - RNA, 20 nt, synthetic construct
  source 1..20: mol_type = other RNA
tgttactgacctatgcgggc

SEQ ID NO: 22715 - RNA, 20 nt, synthetic construct
  source 1..20: mol_type = other RNA
tactgacctatgcgggctgg

SEQ ID NO: 22716 - RNA, 20 nt, synthetic construct
  source 1..20: mol_type = other RNA
actgacctatgcgggctgga

SEQ ID NO: 22717 - RNA, 20 nt, synthetic construct
  source 1..20: mol_type = other RNA
ctgatccctccagcccgcat

SEQ ID NO: 22718 - RNA, 20 nt, synthetic construct
  source 1..20: mol_type = other RNA
ggagggatcagagtagttgc

SEQ ID NO: 22719 - RNA, 20 nt, synthetic construct
  source 1..20: mol_type = other RNA
gttgcaggcatgagatctcc

SEQ ID NO: 22720 - RNA, 20 nt, synthetic construct
  source 1..20: mol_type = other RNA
gcaggcatgagatctcctgg

SEQ ID NO: 22721 - RNA, 20 nt, synthetic construct
  source 1..20: mol_type = other RNA
cttcatctctgttttcctcc

SEQ ID NO: 22722 - RNA, 20 nt, synthetic construct
  source 1..20: mol_type = other RNA
tgctaagttattaacacaca

SEQ ID NO: 22723 - RNA, 20 nt, synthetic construct
  source 1..20: mol_type = other RNA
agaagtgagtgggagcttgg

SEQ ID NO: 22724 - RNA, 20 nt, synthetic construct
  source 1..20: mol_type = other RNA
ctcagaagtgagtgggagct

SEQ ID NO: 22725 - RNA, 20 nt, synthetic construct
  source 1..20: mol_type = other RNA
aaagaatctcagaagtgagt

SEQ ID NO: 22726 - RNA, 20 nt, synthetic construct
  source 1..20: mol_type = other RNA
caaagaatctcagaagtgag

SEQ ID NO: 22727 - RNA, 20 nt, synthetic construct
  source 1..20: mol_type = other RNA
gcctcggcctcccaaagttc

SEQ ID NO: 22728 - RNA, 20 nt, synthetic construct
  source 1..20: mol_type = other RNA
cctcggcctcccaaagttct

SEQ ID NO: 22729 - RNA, 20 nt, synthetic construct
  source 1..20: mol_type = other RNA
gaactttgggaggccgaggc

SEQ ID NO: 22730 - RNA, 20 nt, synthetic construct
  source 1..20: mol_type = other RNA
cccagaactttgggaggccg

SEQ ID NO: 22731 - RNA, 20 nt, synthetic construct
  source 1..20: mol_type = other RNA
tcccaaagttctgggattac

SEQ ID NO: 22732 - RNA, 20 nt, synthetic construct
  source 1..20: mol_type = other RNA
tgtaatcccagaactttggg

SEQ ID NO: 22733 - RNA, 20 nt, synthetic construct
  source 1..20: mol_type = other RNA
gcctgtaatcccagaacttt

SEQ ID NO: 22734 - RNA, 20 nt, synthetic construct
  source 1..20: mol_type = other RNA
cgcctgtaatcccagaactt

SEQ ID NO: 22735 - RNA, 20 nt, synthetic construct
  source 1..20: mol_type = other RNA
aatgaaggagctgggcacag

SEQ ID NO: 22736 - RNA, 20 nt, synthetic construct
  source 1..20: mol_type = other RNA
agaaaatcaatgaaggagct

SEQ ID NO: 22737 - RNA, 20 nt, synthetic construct
  source 1..20: mol_type = other RNA
aagaaaatcaatgaaggagc

SEQ ID NO: 22738 - RNA, 20 nt, synthetic construct
  source 1..20: mol_type = other RNA
aggagaaagaaaatcaatga

SEQ ID NO: 22739 - RNA, 20 nt, synthetic construct
  source 1..20: mol_type = other RNA
cctcccacctctgagttctc

SEQ ID NO: 22740 - RNA, 20 nt, synthetic construct
  source 1..20: mol_type = other RNA
ccagagaactcagaggtggg

SEQ ID NO: 22741 - RNA, 20 nt, synthetic construct
  source 1..20: mol_type = other RNA
attccagagaactcagaggt

SEQ ID NO: 22742 - RNA, 20 nt, synthetic construct
  source 1..20: mol_type = other RNA
aattccagagaactcagagg

SEQ ID NO: 22743 - RNA, 20 nt, synthetic construct
  source 1..20: mol_type = other RNA
tgagttctctggaattgtcc

SEQ ID NO: 22744 - RNA, 20 nt, synthetic construct
  source 1..20: mol_type = other RNA
gacaattccagagaactcag

SEQ ID NO: 22745 - RNA, 20 nt, synthetic construct
  source 1..20: mol_type = other RNA
ggaattgtcctggatttacc

SEQ ID NO: 22746 - RNA, 20 nt, synthetic construct
  source 1..20: mol_type = other RNA
ggatttacctggtttcacca

SEQ ID NO: 22747 - RNA, 20 nt, synthetic construct
  source 1..20: mol_type = other RNA
tggtgaaaccaggtaaatcc

SEQ ID NO: 22748 - RNA, 20 nt, synthetic construct
  source 1..20: mol_type = other RNA
tgggaggccttggtgaaacc

SEQ ID NO: 22749 - RNA, 20 nt, synthetic construct
  source 1..20: mol_type = other RNA
gactctggtgtgggaggcct

SEQ ID NO: 22750 - RNA, 20 nt, synthetic construct
  source 1..20: mol_type = other RNA
agatgagactctggtgtggg

SEQ ID NO: 22751 - RNA, 20 nt, synthetic construct
  source 1..20: mol_type = other RNA
gaaagatgagactctggtgt

SEQ ID NO: 22752 - RNA, 20 nt, synthetic construct
  source 1..20: mol_type = other RNA
agaaagatgagactctggtg

SEQ ID NO: 22753 - RNA, 20 nt, synthetic construct
  source 1..20: mol_type = other RNA
agacaagaaagatgagactc

SEQ ID NO: 22754 - RNA, 20 nt, synthetic construct
  source 1..20: mol_type = other RNA
gcctgatccctgatcccaag

SEQ ID NO: 22755 - RNA, 20 nt, synthetic construct
  source 1..20: mol_type = other RNA
gccacttgggatcagggatc

SEQ ID NO: 22756 - RNA, 20 nt, synthetic construct
  source 1..20: mol_type = other RNA
acgttggccacttgggatca

SEQ ID NO: 22757 - RNA, 20 nt, synthetic construct
  source 1..20: mol_type = other RNA
tacgttggccacttgggatc

SEQ ID NO: 22758 - RNA, 20 nt, synthetic construct
  source 1..20: mol_type = other RNA
gagttctacgttggccactt

SEQ ID NO: 22759 - RNA, 20 nt, synthetic construct
  source 1..20: mol_type = other RNA
ggagttctacgttggccact

SEQ ID NO: 22760 - RNA, 20 nt, synthetic construct
  source 1..20: mol_type = other RNA
cgtagaactccgagaacagc

SEQ ID NO: 22761 - RNA, 20 nt, synthetic construct
  source 1..20: mol_type = other RNA
ctgttctcggagttctacgt

SEQ ID NO: 22762 - RNA, 20 nt, synthetic construct
  source 1..20: mol_type = other RNA
gagaacagctggtcttctcc

SEQ ID NO: 22763 - RNA, 20 nt, synthetic construct
  source 1..20: mol_type = other RNA
agaacagctggtcttctcca

SEQ ID NO: 22764 - RNA, 20 nt, synthetic construct
  source 1..20: mol_type = other RNA
tggagaagaccagctgttct

SEQ ID NO: 22765 - RNA, 20 nt, synthetic construct
  source 1..20: mol_type = other RNA
gagctctgctatcgaagccc

SEQ ID NO: 22766 - RNA, 20 nt, synthetic construct
  source 1..20: mol_type = other RNA
cagagctccagttcctgaag

SEQ ID NO: 22767 - RNA, 20 nt, synthetic construct
  source 1..20: mol_type = other RNA
ctctttgcctcttcaggaac

SEQ ID NO: 22768 - RNA, 20 nt, synthetic construct
  source 1..20: mol_type = other RNA
actcaactctttgcctcttc

SEQ ID NO: 22769 - RNA, 20 nt, synthetic construct
  source 1..20: mol_type = other RNA
gccaccctgttcatcttgca

SEQ ID NO: 22770 - RNA, 20 nt, synthetic construct
  source 1..20: mol_type = other RNA
ccctgttcatcttgcatgga

SEQ ID NO: 22771 - RNA, 20 nt, synthetic construct
  source 1..20: mol_type = other RNA
tccatgcaagatgaacaggg

SEQ ID NO: 22772 - RNA, 20 nt, synthetic construct
  source 1..20: mol_type = other RNA
ccttccatgcaagatgaaca

SEQ ID NO: 22773 - RNA, 20 nt, synthetic construct
  source 1..20: mol_type = other RNA
accttccatgcaagatgaac

SEQ ID NO: 22774 - RNA, 20 nt, synthetic construct
  source 1..20: mol_type = other RNA
ttccccacctgacaccttct

SEQ ID NO: 22775 - RNA, 20 nt, synthetic construct
  source 1..20: mol_type = other RNA
ggccaagaaggtgtcaggtg

SEQ ID NO: 22776 - RNA, 20 nt, synthetic construct
  source 1..20: mol_type = other RNA
gggccaagaaggtgtcaggt

SEQ ID NO: 22777 - RNA, 20 nt, synthetic construct
  source 1..20: mol_type = other RNA
agggccaagaaggtgtcagg

SEQ ID NO: 22778 - RNA, 20 nt, synthetic construct
  source 1..20: mol_type = other RNA
gacaccttcttggccctgct

SEQ ID NO: 22779 - RNA, 20 nt, synthetic construct
  source 1..20: mol_type = other RNA
agcagggccaagaaggtgtc

SEQ ID NO: 22780 - RNA, 20 nt, synthetic construct
  source 1..20: mol_type = other RNA
ggagccaagcagggccaaga

SEQ ID NO: 22781 - RNA, 20 nt, synthetic construct
  source 1..20: mol_type = other RNA
tggccctgcttggctccata

SEQ ID NO: 22782 - RNA, 20 nt, synthetic construct
  source 1..20: mol_type = other RNA
tgtccttatggagccaagca

SEQ ID NO: 22783 - RNA, 20 nt, synthetic construct
  source 1..20: mol_type = other RNA
gtgtccttatggagccaagc

SEQ ID NO: 22784 - RNA, 20 nt, synthetic construct
  source 1..20: mol_type = other RNA
ggatcatcagagtgtcctta

SEQ ID NO: 22785 - RNA, 20 nt, synthetic construct
  source 1..20: mol_type = other RNA
aggttgaacagaaagtgagt

SEQ ID NO: 22786 - RNA, 20 nt, synthetic construct
  source 1..20: mol_type = other RNA
gaggttgaacagaaagtgag

SEQ ID NO: 22787 - RNA, 20 nt, synthetic construct
  source 1..20: mol_type = other RNA
ctcagggacaggataaatcg

SEQ ID NO: 22788 - RNA, 20 nt, synthetic construct
  source 1..20: mol_type = other RNA
ctcagggctttctcagggac

SEQ ID NO: 22789 - RNA, 20 nt, synthetic construct
  source 1..20: mol_type = other RNA
caggtctcagggctttctca

SEQ ID NO: 22790 - RNA, 20 nt, synthetic construct
  source 1..20: mol_type = other RNA
gcaggtctcagggctttctc

SEQ ID NO: 22791 - RNA, 20 nt, synthetic construct
  source 1..20: mol_type = other RNA
agccctgagacctgccccac

SEQ ID NO: 22792 - RNA, 20 nt, synthetic construct
  source 1..20: mol_type = other RNA
tgcctgtggggcaggtctca

SEQ ID NO: 22793 - RNA, 20 nt, synthetic construct
  source 1..20: mol_type = other RNA
atgcctgtggggcaggtctc

SEQ ID NO: 22794 - RNA, 20 nt, synthetic construct
  source 1..20: mol_type = other RNA
ccccacaggcattcattccc

SEQ ID NO: 22795 - RNA, 20 nt, synthetic construct
  source 1..20: mol_type = other RNA
ggaatgaatgcctgtggggc

SEQ ID NO: 22796 - RNA, 20 nt, synthetic construct
  source 1..20: mol_type = other RNA
acaggcattcattcccaggt

SEQ ID NO: 22797 - RNA, 20 nt, synthetic construct
  source 1..20: mol_type = other RNA
cctgggaatgaatgcctgtg

SEQ ID NO: 22798 - RNA, 20 nt, synthetic construct
  source 1..20: mol_type = other RNA
acctgggaatgaatgcctgt

SEQ ID NO: 22799 - RNA, 20 nt, synthetic construct
  source 1..20: mol_type = other RNA
tacctgggaatgaatgcctg

SEQ ID NO: 22800 - RNA, 20 nt, synthetic construct
  source 1..20: mol_type = other RNA
tgcgaacagaagtcctacct

SEQ ID NO: 22801 - RNA, 20 nt, synthetic construct
  source 1..20: mol_type = other RNA
ctgcgaacagaagtcctacc

SEQ ID NO: 22802 - RNA, 20 nt, synthetic construct
  source 1..20: mol_type = other RNA
gacttctgttcgcagtgaag

SEQ ID NO: 22803 - RNA, 20 nt, synthetic construct
  source 1..20: mol_type = other RNA
cgcagtgaagaggcagacac

SEQ ID NO: 22804 - RNA, 20 nt, synthetic construct
  source 1..20: mol_type = other RNA
gcagtgaagaggcagacact

SEQ ID NO: 22805 - RNA, 20 nt, synthetic construct
  source 1..20: mol_type = other RNA
agacactgggctgctcacct

SEQ ID NO: 22806 - RNA, 20 nt, synthetic construct
  source 1..20: mol_type = other RNA
gacactgggctgctcacctt

SEQ ID NO: 22807 - RNA, 20 nt, synthetic construct
  source 1..20: mol_type = other RNA
acactgggctgctcaccttg

SEQ ID NO: 22808 - RNA, 20 nt, synthetic construct
  source 1..20: mol_type = other RNA
gatgctggaaatactcccca

SEQ ID NO: 22809 - RNA, 20 nt, synthetic construct
  source 1..20: mol_type = other RNA
tgggtctggttcagggatgc

SEQ ID NO: 22810 - RNA, 20 nt, synthetic construct
  source 1..20: mol_type = other RNA
ctgtgtctgggtctggttca

SEQ ID NO: 22811 - RNA, 20 nt, synthetic construct
  source 1..20: mol_type = other RNA
actgtgtctgggtctggttc

SEQ ID NO: 22812 - RNA, 20 nt, synthetic construct
  source 1..20: mol_type = other RNA
cgttacactgtgtctgggtc

SEQ ID NO: 22813 - RNA, 20 nt, synthetic construct
  source 1..20: mol_type = other RNA
gctgtcgttacactgtgtct

SEQ ID NO: 22814 - RNA, 20 nt, synthetic construct
  source 1..20: mol_type = other RNA
ggctgtcgttacactgtgtc

SEQ ID NO: 22815 - RNA, 20 nt, synthetic construct
  source 1..20: mol_type = other RNA
taacgacagcccatataaag

SEQ ID NO: 22816 - RNA, 20 nt, synthetic construct
  source 1..20: mol_type = other RNA
aacgacagcccatataaagt

SEQ ID NO: 22817 - RNA, 20 nt, synthetic construct
  source 1..20: mol_type = other RNA
acgacagcccatataaagtg

SEQ ID NO: 22818 - RNA, 20 nt, synthetic construct
  source 1..20: mol_type = other RNA
cccatataaagtggggtcag

SEQ ID NO: 22819 - RNA, 20 nt, synthetic construct
  source 1..20: mol_type = other RNA
ccatataaagtggggtcagc

SEQ ID NO: 22820 - RNA, 20 nt, synthetic construct
  source 1..20: mol_type = other RNA
catataaagtggggtcagcg

SEQ ID NO: 22821 - RNA, 20 nt, synthetic construct
  source 1..20: mol_type = other RNA
atataaagtggggtcagcgg

SEQ ID NO: 22822 - RNA, 20 nt, synthetic construct
  source 1..20: mol_type = other RNA
ccgctgaccccactttatat

SEQ ID NO: 22823 - RNA, 20 nt, synthetic construct
  source 1..20: mol_type = other RNA
taaagtggggtcagcggggg

SEQ ID NO: 22824 - RNA, 20 nt, synthetic construct
  source 1..20: mol_type = other RNA
gggtcagcgggggtggcttg

SEQ ID NO: 22825 - RNA, 20 nt, synthetic construct
  source 1..20: mol_type = other RNA
gcttgtggattcgcacaaac

SEQ ID NO: 22826 - RNA, 20 nt, synthetic construct
  source 1..20: mol_type = other RNA
tttcatttctagatcatcta

SEQ ID NO: 22827 - RNA, 20 nt, synthetic construct
  source 1..20: mol_type = other RNA
atctatggcctacagaacat

SEQ ID NO: 22828 - RNA, 20 nt, synthetic construct
  source 1..20: mol_type = other RNA
tctatggcctacagaacata

SEQ ID NO: 22829 - RNA, 20 nt, synthetic construct
  source 1..20: mol_type = other RNA
cattgttccctatgttctgt

SEQ ID NO: 22830 - RNA, 20 nt, synthetic construct
  source 1..20: mol_type = other RNA
aacatagggaacaatgatta

SEQ ID NO: 22831 - RNA, 20 nt, synthetic construct
  source 1..20: mol_type = other RNA
acatagggaacaatgattaa

SEQ ID NO: 22832 - RNA, 20 nt, synthetic construct
  source 1..20: mol_type = other RNA
tagggaacaatgattaaggg

SEQ ID NO: 22833 - RNA, 20 nt, synthetic construct
  source 1..20: mol_type = other RNA
taagggaggcttctgccccg

SEQ ID NO: 22834 - RNA, 20 nt, synthetic construct
  source 1..20: mol_type = other RNA
ggcttctgccccgtggaatg

SEQ ID NO: 22835 - RNA, 20 nt, synthetic construct
  source 1..20: mol_type = other RNA
ccgtggaatgtggtttgaat

SEQ ID NO: 22836 - RNA, 20 nt, synthetic construct
  source 1..20: mol_type = other RNA
cgtggaatgtggtttgaata

SEQ ID NO: 22837 - RNA, 20 nt, synthetic construct
  source 1..20: mol_type = other RNA
gtggaatgtggtttgaatag

SEQ ID NO: 22838 - RNA, 20 nt, synthetic construct
  source 1..20: mol_type = other RNA
tggaatgtggtttgaatagg

SEQ ID NO: 22839 - RNA, 20 nt, synthetic construct
  source 1..20: mol_type = other RNA
ggaatgtggtttgaataggg

SEQ ID NO: 22840 - RNA, 20 nt, synthetic construct
  source 1..20: mol_type = other RNA
cctattcaaaccacattcca

SEQ ID NO: 22841 - RNA, 20 nt, synthetic construct
  source 1..20: mol_type = other RNA
tgtggtttgaatagggggga

SEQ ID NO: 22842 - RNA, 20 nt, synthetic construct
  source 1..20: mol_type = other RNA
ggtgcatctgtgtgtttgtg

SEQ ID NO: 22843 - RNA, 20 nt, synthetic construct
  source 1..20: mol_type = other RNA
gtgtgtttgtgtggacagag

SEQ ID NO: 22844 - RNA, 20 nt, synthetic construct
  source 1..20: mol_type = other RNA
tgtgtttgtgtggacagagt

SEQ ID NO: 22845 - RNA, 20 nt, synthetic construct
  source 1..20: mol_type = other RNA
gtgtttgtgtggacagagtg

SEQ ID NO: 22846 - RNA, 20 nt, synthetic construct
  source 1..20: mol_type = other RNA
ctgtacaagaggcccatcct

SEQ ID NO: 22847 - RNA, 20 nt, synthetic construct
  source 1..20: mol_type = other RNA
caaggatgggcctcttgtac

SEQ ID NO: 22848 - RNA, 20 nt, synthetic construct
  source 1..20: mol_type = other RNA
cttcaactgggaccaaggat

SEQ ID NO: 22849 - RNA, 20 nt, synthetic construct
  source 1..20: mol_type = other RNA
tcttcaactgggaccaagga

SEQ ID NO: 22850 - RNA, 20 nt, synthetic construct
  source 1..20: mol_type = other RNA
gtcccagttgaagaccctct

SEQ ID NO: 22851 - RNA, 20 nt, synthetic construct
  source 1..20: mol_type = other RNA
tcccagttgaagaccctcta

SEQ ID NO: 22852 - RNA, 20 nt, synthetic construct
  source 1..20: mol_type = other RNA
cccagttgaagaccctctag

SEQ ID NO: 22853 - RNA, 20 nt, synthetic construct
  source 1..20: mol_type = other RNA
ccagttgaagaccctctagg

SEQ ID NO: 22854 - RNA, 20 nt, synthetic construct
  source 1..20: mol_type = other RNA
cccctagagggtcttcaact

SEQ ID NO: 22855 - RNA, 20 nt, synthetic construct
  source 1..20: mol_type = other RNA
ccccctagagggtcttcaac

SEQ ID NO: 22856 - RNA, 20 nt, synthetic construct
  source 1..20: mol_type = other RNA
agaccctctagggggctctc

SEQ ID NO: 22857 - RNA, 20 nt, synthetic construct
  source 1..20: mol_type = other RNA
cagccagagagccccctaga

SEQ ID NO: 22858 - RNA, 20 nt, synthetic construct
  source 1..20: mol_type = other RNA
gcagccagagagccccctag

SEQ ID NO: 22859 - RNA, 20 nt, synthetic construct
  source 1..20: mol_type = other RNA
tgtttaccgtcaacccaccg

SEQ ID NO: 22860 - RNA, 20 nt, synthetic construct
  source 1..20: mol_type = other RNA
gctgggccacggtgggttga

SEQ ID NO: 22861 - RNA, 20 nt, synthetic construct
  source 1..20: mol_type = other RNA
ccaccgtggcccagcctttc

SEQ ID NO: 22862 - RNA, 20 nt, synthetic construct
  source 1..20: mol_type = other RNA
cagaaaggctgggccacggt

SEQ ID NO: 22863 - RNA, 20 nt, synthetic construct
  source 1..20: mol_type = other RNA
ccagaaaggctgggccacgg

SEQ ID NO: 22864 - RNA, 20 nt, synthetic construct
  source 1..20: mol_type = other RNA
gagccagaaaggctgggcca

SEQ ID NO: 22865 - RNA, 20 nt, synthetic construct
  source 1..20: mol_type = other RNA
cactaagagccagaaaggct

SEQ ID NO: 22866 - RNA, 20 nt, synthetic construct
  source 1..20: mol_type = other RNA
acactaagagccagaaaggc

SEQ ID NO: 22867 - RNA, 20 nt, synthetic construct
  source 1..20: mol_type = other RNA
ggtgacactaagagccagaa

SEQ ID NO: 22868 - RNA, 20 nt, synthetic construct
  source 1..20: mol_type = other RNA
tcttagtgtcaccttccgaa

SEQ ID NO: 22869 - RNA, 20 nt, synthetic construct
  source 1..20: mol_type = other RNA
ttccgaatggagcagtcact

SEQ ID NO: 22870 - RNA, 20 nt, synthetic construct
  source 1..20: mol_type = other RNA
tccgaatggagcagtcactt

SEQ ID NO: 22871 - RNA, 20 nt, synthetic construct
  source 1..20: mol_type = other RNA
aagtgactgctccattcgga

SEQ ID NO: 22872 - RNA, 20 nt, synthetic construct
  source 1..20: mol_type = other RNA
tggagcagtcacttgggatc

SEQ ID NO: 22873 - RNA, 20 nt, synthetic construct
  source 1..20: mol_type = other RNA
agtcacttgggatcaggtag

SEQ ID NO: 22874 - RNA, 20 nt, synthetic construct
  source 1..20: mol_type = other RNA
cacttgggatcaggtagagg

SEQ ID NO: 22875 - RNA, 20 nt, synthetic construct
  source 1..20: mol_type = other RNA
tgggatcaggtagaggtgga

SEQ ID NO: 22876 - RNA, 20 nt, synthetic construct
  source 1..20: mol_type = other RNA
aggtggaaggtgacttcctc

SEQ ID NO: 22877 - RNA, 20 nt, synthetic construct
  source 1..20: mol_type = other RNA
ggaaggtgacttcctcagga

SEQ ID NO: 22878 - RNA, 20 nt, synthetic construct
  source 1..20: mol_type = other RNA
tgacttcctcaggatggacg

SEQ ID NO: 22879 - RNA, 20 nt, synthetic construct
  source 1..20: mol_type = other RNA
cttcctcaggatggacgcgg

SEQ ID NO: 22880 - RNA, 20 nt, synthetic construct
  source 1..20: mol_type = other RNA
ttaccaccgcgtccatcctg

SEQ ID NO: 22881 - RNA, 20 nt, synthetic construct
  source 1..20: mol_type = other RNA
gtggtaaagcaacaccacag

SEQ ID NO: 22882 - RNA, 20 nt, synthetic construct
  source 1..20: mol_type = other RNA
aagcaacaccacagaggtga

SEQ ID NO: 22883 - RNA, 20 nt, synthetic construct
  source 1..20: mol_type = other RNA
agcaacaccacagaggtgac

SEQ ID NO: 22884 - RNA, 20 nt, synthetic construct
  source 1..20: mol_type = other RNA
cttcattcccgtcacctctg

SEQ ID NO: 22885 - RNA, 20 nt, synthetic construct
  source 1..20: mol_type = other RNA
aggtgacgggaatgaagcgc

SEQ ID NO: 22886 - RNA, 20 nt, synthetic construct
  source 1..20: mol_type = other RNA
ggtgacgggaatgaagcgca

SEQ ID NO: 22887 - RNA, 20 nt, synthetic construct
  source 1..20: mol_type = other RNA
gaatgaagcgcagggcatta

SEQ ID NO: 22888 - RNA, 20 nt, synthetic construct
  source 1..20: mol_type = other RNA
gggcattatggatcattttc

SEQ ID NO: 22889 - RNA, 20 nt, synthetic construct
  source 1..20: mol_type = other RNA
cattatggatcattttcagg

SEQ ID NO: 22890 - RNA, 20 nt, synthetic construct
  source 1..20: mol_type = other RNA
cattttcaggaggactccca

SEQ ID NO: 22891 - RNA, 20 nt, synthetic construct
  source 1..20: mol_type = other RNA
attttcaggaggactcccaa

SEQ ID NO: 22892 - RNA, 20 nt, synthetic construct
  source 1..20: mol_type = other RNA
ttttcaggaggactcccaag

SEQ ID NO: 22893 - RNA, 20 nt, synthetic construct
  source 1..20: mol_type = other RNA
tttcaggaggactcccaagg

SEQ ID NO: 22894 - RNA, 20 nt, synthetic construct
  source 1..20: mol_type = other RNA
gactcccaagggggagaagc

SEQ ID NO: 22895 - RNA, 20 nt, synthetic construct
  source 1..20: mol_type = other RNA
actcccaagggggagaagct

SEQ ID NO: 22896 - RNA, 20 nt, synthetic construct
  source 1..20: mol_type = other RNA
ctcccaagggggagaagctg

SEQ ID NO: 22897 - RNA, 20 nt, synthetic construct
  source 1..20: mol_type = other RNA
aaccccagcttctccccctt

SEQ ID NO: 22898 - RNA, 20 nt, synthetic construct
  source 1..20: mol_type = other RNA
aaaccccagcttctccccct

SEQ ID NO: 22899 - RNA, 20 nt, synthetic construct
  source 1..20: mol_type = other RNA
ggagctgcatcacatagttc

SEQ ID NO: 22900 - RNA, 20 nt, synthetic construct
  source 1..20: mol_type = other RNA
tatgtgatgcagctccaccc

SEQ ID NO: 22901 - RNA, 20 nt, synthetic construct
  source 1..20: mol_type = other RNA
tgatgcagctccaccctggc

SEQ ID NO: 22902 - RNA, 20 nt, synthetic construct
  source 1..20: mol_type = other RNA
ccaccctggctggcttctcc

SEQ ID NO: 22903 - RNA, 20 nt, synthetic construct
  source 1..20: mol_type = other RNA
cctggagaagccagccaggg

SEQ ID NO: 22904 - RNA, 20 nt, synthetic construct
  source 1..20: mol_type = other RNA
gctcctggagaagccagcca

SEQ ID NO: 22905 - RNA, 20 nt, synthetic construct
  source 1..20: mol_type = other RNA
tgctcctggagaagccagcc

SEQ ID NO: 22906 - RNA, 20 nt, synthetic construct
  source 1..20: mol_type = other RNA
taaagaggaggggatgctcc

SEQ ID NO: 22907 - RNA, 20 nt, synthetic construct
  source 1..20: mol_type = other RNA
gcatcccctcctctttaaag

SEQ ID NO: 22908 - RNA, 20 nt, synthetic construct
  source 1..20: mol_type = other RNA
catcccctcctctttaaagt

SEQ ID NO: 22909 - RNA, 20 nt, synthetic construct
  source 1..20: mol_type = other RNA
cctctttaaagtgggccatt

SEQ ID NO: 22910 - RNA, 20 nt, synthetic construct
  source 1..20: mol_type = other RNA
atggcccactttaaagagga

SEQ ID NO: 22911 - RNA, 20 nt, synthetic construct
  source 1..20: mol_type = other RNA
aatggcccactttaaagagg

SEQ ID NO: 22912 - RNA, 20 nt, synthetic construct
  source 1..20: mol_type = other RNA
ccaaatggcccactttaaag

SEQ ID NO: 22913 - RNA, 20 nt, synthetic construct
  source 1..20: mol_type = other RNA
taaagtgggccatttggaac

SEQ ID NO: 22914 - RNA, 20 nt, synthetic construct
  source 1..20: mol_type = other RNA
aaagtgggccatttggaaca

SEQ ID NO: 22915 - RNA, 20 nt, synthetic construct
  source 1..20: mol_type = other RNA
ggacacatccctgttccaaa

SEQ ID NO: 22916 - RNA, 20 nt, synthetic construct
  source 1..20: mol_type = other RNA
ggaacagggatgtgtccaca

SEQ ID NO: 22917 - RNA, 20 nt, synthetic construct
  source 1..20: mol_type = other RNA
catggccccctgtaaaagaa

SEQ ID NO: 22918 - RNA, 20 nt, synthetic construct
  source 1..20: mol_type = other RNA
ttcttttacagggggccatg

SEQ ID NO: 22919 - RNA, 20 nt, synthetic construct
  source 1..20: mol_type = other RNA
tcaatccattcttttacagg

SEQ ID NO: 22920 - RNA, 20 nt, synthetic construct
  source 1..20: mol_type = other RNA
ttcaatccattcttttacag

SEQ ID NO: 22921 - RNA, 20 nt, synthetic construct
  source 1..20: mol_type = other RNA
cttcaatccattcttttaca

SEQ ID NO: 22922 - RNA, 20 nt, synthetic construct
  source 1..20: mol_type = other RNA
tcttcaatccattcttttac

SEQ ID NO: 22923 - RNA, 20 nt, synthetic construct
  source 1..20: mol_type = other RNA
agaatggattgaagaggcac

SEQ ID NO: 22924 - RNA, 20 nt, synthetic construct
  source 1..20: mol_type = other RNA
gagtttcgctcttgtcgccc

SEQ ID NO: 22925 - RNA, 20 nt, synthetic construct
  source 1..20: mol_type = other RNA
ttcgctcttgtcgcccaggc

SEQ ID NO: 22926 - RNA, 20 nt, synthetic construct
  source 1..20: mol_type = other RNA
tcgcccaggctggagtgcaa

SEQ ID NO: 22927 - RNA, 20 nt, synthetic construct
  source 1..20: mol_type = other RNA
gtaccattgcactccagcct

SEQ ID NO: 22928 - RNA, 20 nt, synthetic construct
  source 1..20: mol_type = other RNA
tgtaccattgcactccagcc

SEQ ID NO: 22929 - RNA, 20 nt, synthetic construct
  source 1..20: mol_type = other RNA
ggagtgcaatggtacaatct

SEQ ID NO: 22930 - RNA, 20 nt, synthetic construct
  source 1..20: mol_type = other RNA
gaggggccgagggggggtta

SEQ ID NO: 22931 - RNA, 20 nt, synthetic construct
  source 1..20: mol_type = other RNA
tccttagaggggccgagggg

SEQ ID NO: 22932 - RNA, 20 nt, synthetic construct
  source 1..20: mol_type = other RNA
ttccttagaggggccgaggg

SEQ ID NO: 22933 - RNA, 20 nt, synthetic construct
  source 1..20: mol_type = other RNA
cttccttagaggggccgagg

SEQ ID NO: 22934 - RNA, 20 nt, synthetic construct
  source 1..20: mol_type = other RNA
gcttccttagaggggccgag

SEQ ID NO: 22935 - RNA, 20 nt, synthetic construct
  source 1..20: mol_type = other RNA
ggcttccttagaggggccga

SEQ ID NO: 22936 - RNA, 20 nt, synthetic construct
  source 1..20: mol_type = other RNA
tggcttccttagaggggccg

SEQ ID NO: 22937 - RNA, 20 nt, synthetic construct
  source 1..20: mol_type = other RNA
gtgttgtggcttccttagag

SEQ ID NO: 22938 - RNA, 20 nt, synthetic construct
  source 1..20: mol_type = other RNA
ggtgttgtggcttccttaga

SEQ ID NO: 22939 - RNA, 20 nt, synthetic construct
  source 1..20: mol_type = other RNA
gggtgttgtggcttccttag

SEQ ID NO: 22940 - RNA, 20 nt, synthetic construct
  source 1..20: mol_type = other RNA
aagccacaacaccctctccc

SEQ ID NO: 22941 - RNA, 20 nt, synthetic construct
  source 1..20: mol_type = other RNA
tctcctgggagagggtgttg

SEQ ID NO: 22942 - RNA, 20 nt, synthetic construct
  source 1..20: mol_type = other RNA
aatgataatctcctgggaga

SEQ ID NO: 22943 - RNA, 20 nt, synthetic construct
  source 1..20: mol_type = other RNA
gaatgataatctcctgggag

SEQ ID NO: 22944 - RNA, 20 nt, synthetic construct
  source 1..20: mol_type = other RNA
gtgtagaatgataatctcct

SEQ ID NO: 22945 - RNA, 20 nt, synthetic construct
  source 1..20: mol_type = other RNA
agtgtagaatgataatctcc

SEQ ID NO: 22946 - RNA, 20 nt, synthetic construct
  source 1..20: mol_type = other RNA
atcattctacactccctttc

SEQ ID NO: 22947 - RNA, 20 nt, synthetic construct
  source 1..20: mol_type = other RNA
tggtaattatgggcctgaaa

SEQ ID NO: 22948 - RNA, 20 nt, synthetic construct
  source 1..20: mol_type = other RNA
gtggtaattatgggcctgaa

SEQ ID NO: 22949 - RNA, 20 nt, synthetic construct
  source 1..20: mol_type = other RNA
aggaaggtggtggtaattat

SEQ ID NO: 22950 - RNA, 20 nt, synthetic construct
  source 1..20: mol_type = other RNA
gaggaaggtggtggtaatta

SEQ ID NO: 22951 - RNA, 20 nt, synthetic construct
  source 1..20: mol_type = other RNA
aaggatagggaggaaggtgg

SEQ ID NO: 22952 - RNA, 20 nt, synthetic construct
  source 1..20: mol_type = other RNA
gggaaggatagggaggaagg

SEQ ID NO: 22953 - RNA, 20 nt, synthetic construct
  source 1..20: mol_type = other RNA
acagggaaggatagggagga

SEQ ID NO: 22954 - RNA, 20 nt, synthetic construct
  source 1..20: mol_type = other RNA
aacaacagggaaggataggg

SEQ ID NO: 22955 - RNA, 20 nt, synthetic construct
  source 1..20: mol_type = other RNA
gtaaacaacagggaaggata

SEQ ID NO: 22956 - RNA, 20 nt, synthetic construct
  source 1..20: mol_type = other RNA
ggtaaacaacagggaaggat

SEQ ID NO: 22957 - RNA, 20 nt, synthetic construct
  source 1..20: mol_type = other RNA
tccaaggtaaacaacaggga

SEQ ID NO: 22958 - RNA, 20 nt, synthetic construct
  source 1..20: mol_type = other RNA
gctctccaaggtaaacaaca

SEQ ID NO: 22959 - RNA, 20 nt, synthetic construct
  source 1..20: mol_type = other RNA
ggctctccaaggtaaacaac

SEQ ID NO: 22960 - RNA, 20 nt, synthetic construct
  source 1..20: mol_type = other RNA
ccttggagagccacaaagtg

SEQ ID NO: 22961 - RNA, 20 nt, synthetic construct
  source 1..20: mol_type = other RNA
cttggagagccacaaagtga

SEQ ID NO: 22962 - RNA, 20 nt, synthetic construct
  source 1..20: mol_type = other RNA
ggagagccacaaagtgaggg

SEQ ID NO: 22963 - RNA, 20 nt, synthetic construct
  source 1..20: mol_type = other RNA
cctcactttgtggctctcca

SEQ ID NO: 22964 - RNA, 20 nt, synthetic construct
  source 1..20: mol_type = other RNA
tgtgcacctccctcactttg

SEQ ID NO: 22965 - RNA, 20 nt, synthetic construct
  source 1..20: mol_type = other RNA
tgcacagcttccacagctcc

SEQ ID NO: 22966 - RNA, 20 nt, synthetic construct
  source 1..20: mol_type = other RNA
caaggctgagcctggagctg

SEQ ID NO: 22967 - RNA, 20 nt, synthetic construct
  source 1..20: mol_type = other RNA
ctggacatcaaggctgagcc

SEQ ID NO: 22968 - RNA, 20 nt, synthetic construct
  source 1..20: mol_type = other RNA
tcagccttgatgtccagcag

SEQ ID NO: 22969 - RNA, 20 nt, synthetic construct
  source 1..20: mol_type = other RNA
agggcctctgctggacatca

SEQ ID NO: 22970 - RNA, 20 nt, synthetic construct
  source 1..20: mol_type = other RNA
gatggtggcagggcctctgc

SEQ ID NO: 22971 - RNA, 20 nt, synthetic construct
  source 1..20: mol_type = other RNA
gccaccatccagctgtgctg

SEQ ID NO: 22972 - RNA, 20 nt, synthetic construct
  source 1..20: mol_type = other RNA
agcacagctggatggtggca

SEQ ID NO: 22973 - RNA, 20 nt, synthetic construct
  source 1..20: mol_type = other RNA
cagcacagctggatggtggc

SEQ ID NO: 22974 - RNA, 20 nt, synthetic construct
  source 1..20: mol_type = other RNA
cccacagcacagctggatgg

SEQ ID NO: 22975 - RNA, 20 nt, synthetic construct
  source 1..20: mol_type = other RNA
caacccacagcacagctgga

SEQ ID NO: 22976 - RNA, 20 nt, synthetic construct
  source 1..20: mol_type = other RNA
agatcaacccacagcacagc

SEQ ID NO: 22977 - RNA, 20 nt, synthetic construct
  source 1..20: mol_type = other RNA
gctgtgggttgatctcaccc

SEQ ID NO: 22978 - RNA, 20 nt, synthetic construct
  source 1..20: mol_type = other RNA
ggttgatctcacccaggaac

SEQ ID NO: 22979 - RNA, 20 nt, synthetic construct
  source 1..20: mol_type = other RNA
tgtgtgtgggaccagttcct

SEQ ID NO: 22980 - RNA, 20 nt, synthetic construct
  source 1..20: mol_type = other RNA
ctgtgtgtgggaccagttcc

SEQ ID NO: 22981 - RNA, 20 nt, synthetic construct
  source 1..20: mol_type = other RNA
cacacagaattcaatctcaa

SEQ ID NO: 22982 - RNA, 20 nt, synthetic construct
  source 1..20: mol_type = other RNA
tgagattgaattctgtgtgt

SEQ ID NO: 22983 - RNA, 20 nt, synthetic construct
  source 1..20: mol_type = other RNA
ttgagattgaattctgtgtg

SEQ ID NO: 22984 - RNA, 20 nt, synthetic construct
  source 1..20: mol_type = other RNA
ctgctttgtgatgagagaag

SEQ ID NO: 22985 - RNA, 20 nt, synthetic construct
  source 1..20: mol_type = other RNA
cacaaagcagagacccgtgt

SEQ ID NO: 22986 - RNA, 20 nt, synthetic construct
  source 1..20: mol_type = other RNA
acaaagcagagacccgtgtt

SEQ ID NO: 22987 - RNA, 20 nt, synthetic construct
  source 1..20: mol_type = other RNA
agagacccgtgttgggccag

SEQ ID NO: 22988 - RNA, 20 nt, synthetic construct
  source 1..20: mol_type = other RNA
acccgtgttgggccagcggt

SEQ ID NO: 22989 - RNA, 20 nt, synthetic construct
  source 1..20: mol_type = other RNA
tcctaccgctggcccaacac

SEQ ID NO: 22990 - RNA, 20 nt, synthetic construct
  source 1..20: mol_type = other RNA
ctcctaccgctggcccaaca

SEQ ID NO: 22991 - RNA, 20 nt, synthetic construct
  source 1..20: mol_type = other RNA
cagcggtaggagccagctac

SEQ ID NO: 22992 - RNA, 20 nt, synthetic construct
  source 1..20: mol_type = other RNA
agcggtaggagccagctaca

SEQ ID NO: 22993 - RNA, 20 nt, synthetic construct
  source 1..20: mol_type = other RNA
ctgtagctggctcctaccgc

SEQ ID NO: 22994 - RNA, 20 nt, synthetic construct
  source 1..20: mol_type = other RNA
agctacagggaagtgaactc

SEQ ID NO: 22995 - RNA, 20 nt, synthetic construct
  source 1..20: mol_type = other RNA
gctacagggaagtgaactct

SEQ ID NO: 22996 - RNA, 20 nt, synthetic construct
  source 1..20: mol_type = other RNA
agagttcacttccctgtagc

SEQ ID NO: 22997 - RNA, 20 nt, synthetic construct
  source 1..20: mol_type = other RNA
aagtgaactctgggaagaag

SEQ ID NO: 22998 - RNA, 20 nt, synthetic construct
  source 1..20: mol_type = other RNA
agtgaactctgggaagaaga

SEQ ID NO: 22999 - RNA, 20 nt, synthetic construct
  source 1..20: mol_type = other RNA
actctgggaagaagagggag

SEQ ID NO: 23000 - RNA, 20 nt, synthetic construct
  source 1..20: mol_type = other RNA
cgaactcactgagcacctgc

SEQ ID NO: 23001 - RNA, 20 nt, synthetic construct
  source 1..20: mol_type = other RNA
ctggatgccagaccccatgc

SEQ ID NO: 23002 - RNA, 20 nt, synthetic construct
  source 1..20: mol_type = other RNA
tggatgccagaccccatgca

SEQ ID NO: 23003 - RNA, 20 nt, synthetic construct
  source 1..20: mol_type = other RNA
ggatgccagaccccatgcag

SEQ ID NO: 23004 - RNA, 20 nt, synthetic construct
  source 1..20: mol_type = other RNA
agaccccatgcaggggcttg

SEQ ID NO: 23005 - RNA, 20 nt, synthetic construct
  source 1..20: mol_type = other RNA
gcaagcccctgcatggggtc

SEQ ID NO: 23006 - RNA, 20 nt, synthetic construct
  source 1..20: mol_type = other RNA
catgcaggggcttgcggata

SEQ ID NO: 23007 - RNA, 20 nt, synthetic construct
  source 1..20: mol_type = other RNA
tatccgcaagcccctgcatg

SEQ ID NO: 23008 - RNA, 20 nt, synthetic construct
  source 1..20: mol_type = other RNA
gtatccgcaagcccctgcat

SEQ ID NO: 23009 - RNA, 20 nt, synthetic construct
  source 1..20: mol_type = other RNA
cgtatccgcaagcccctgca

SEQ ID NO: 23010 - RNA, 20 nt, synthetic construct
  source 1..20: mol_type = other RNA
ggcttgcggatacggtacag

SEQ ID NO: 23011 - RNA, 20 nt, synthetic construct
  source 1..20: mol_type = other RNA
gtggcttcaagcccagactt

SEQ ID NO: 23012 - RNA, 20 nt, synthetic construct
  source 1..20: mol_type = other RNA
acccagtggtgagtgtgagt

SEQ ID NO: 23013 - RNA, 20 nt, synthetic construct
  source 1..20: mol_type = other RNA
cccagtggtgagtgtgagtt

SEQ ID NO: 23014 - RNA, 20 nt, synthetic construct
  source 1..20: mol_type = other RNA
ccagtggtgagtgtgagttg

SEQ ID NO: 23015 - RNA, 20 nt, synthetic construct
  source 1..20: mol_type = other RNA
cagtggtgagtgtgagttgg

SEQ ID NO: 23016 - RNA, 20 nt, synthetic construct
  source 1..20: mol_type = other RNA
cccaactcacactcaccact

SEQ ID NO: 23017 - RNA, 20 nt, synthetic construct
  source 1..20: mol_type = other RNA
ggtgagtgtgagttgggggt

SEQ ID NO: 23018 - RNA, 20 nt, synthetic construct
  source 1..20: mol_type = other RNA
gtgagtgtgagttgggggta

SEQ ID NO: 23019 - RNA, 20 nt, synthetic construct
  source 1..20: mol_type = other RNA
tgagtgtgagttgggggtag

SEQ ID NO: 23020 - RNA, 20 nt, synthetic construct
  source 1..20: mol_type = other RNA
gagtgtgagttgggggtagg

SEQ ID NO: 23021 - RNA, 20 nt, synthetic construct
  source 1..20: mol_type = other RNA
tgtgagttgggggtaggggg

SEQ ID NO: 23022 - RNA, 20 nt, synthetic construct
  source 1..20: mol_type = other RNA
ggggtggcgctgactgtctg

SEQ ID NO: 23023 - RNA, 20 nt, synthetic construct
  source 1..20: mol_type = other RNA
gggtggcgctgactgtctgt

SEQ ID NO: 23024 - RNA, 20 nt, synthetic construct
  source 1..20: mol_type = other RNA
ggtggcgctgactgtctgtg

SEQ ID NO: 23025 - RNA, 20 nt, synthetic construct
  source 1..20: mol_type = other RNA
ctgactgtctgtggggaccc

SEQ ID NO: 23026 - RNA, 20 nt, synthetic construct
  source 1..20: mol_type = other RNA
ctgtctgtggggacccagga

SEQ ID NO: 23027 - RNA, 20 nt, synthetic construct
  source 1..20: mol_type = other RNA
tgtctgtggggacccaggat

SEQ ID NO: 23028 - RNA, 20 nt, synthetic construct
  source 1..20: mol_type = other RNA
tggggacccaggatgggcag

SEQ ID NO: 23029 - RNA, 20 nt, synthetic construct
  source 1..20: mol_type = other RNA
ggggacccaggatgggcagt

SEQ ID NO: 23030 - RNA, 20 nt, synthetic construct
  source 1..20: mol_type = other RNA
gggacccaggatgggcagtg

SEQ ID NO: 23031 - RNA, 20 nt, synthetic construct
  source 1..20: mol_type = other RNA
ccaggatgggcagtggggtg

SEQ ID NO: 23032 - RNA, 20 nt, synthetic construct
  source 1..20: mol_type = other RNA
caggatgggcagtggggtgc

SEQ ID NO: 23033 - RNA, 20 nt, synthetic construct
  source 1..20: mol_type = other RNA
gatgggcagtggggtgcggg

SEQ ID NO: 23034 - RNA, 20 nt, synthetic construct
  source 1..20: mol_type = other RNA
ccgcaccccactgcccatcc

SEQ ID NO: 23035 - RNA, 20 nt, synthetic construct
  source 1..20: mol_type = other RNA
tggggtgcgggaggccagcc

SEQ ID NO: 23036 - RNA, 20 nt, synthetic construct
  source 1..20: mol_type = other RNA
ggggtgcgggaggccagcct

SEQ ID NO: 23037 - RNA, 20 nt, synthetic construct
  source 1..20: mol_type = other RNA
gggctctgctggtcccaggc

SEQ ID NO: 23038 - RNA, 20 nt, synthetic construct
  source 1..20: mol_type = other RNA
gagggggctctgctggtccc

SEQ ID NO: 23039 - RNA, 20 nt, synthetic construct
  source 1..20: mol_type = other RNA
agcagagccccctcactcac

SEQ ID NO: 23040 - RNA, 20 nt, synthetic construct
  source 1..20: mol_type = other RNA
ggtgagtgagggggctctgc

SEQ ID NO: 23041 - RNA, 20 nt, synthetic construct
  source 1..20: mol_type = other RNA
acttgtaccggtgagtgagg

SEQ ID NO: 23042 - RNA, 20 nt, synthetic construct
  source 1..20: mol_type = other RNA
aacttgtaccggtgagtgag

SEQ ID NO: 23043 - RNA, 20 nt, synthetic construct
  source 1..20: mol_type = other RNA
gaacttgtaccggtgagtga

SEQ ID NO: 23044 - RNA, 20 nt, synthetic construct
  source 1..20: mol_type = other RNA
agaacttgtaccggtgagtg

SEQ ID NO: 23045 - RNA, 20 nt, synthetic construct
  source 1..20: mol_type = other RNA
acaaagaaaagaacttgtac

SEQ ID NO: 23046 - RNA, 20 nt, synthetic construct
  source 1..20: mol_type = other RNA
tcaactacctcagtagccac

SEQ ID NO: 23047 - RNA, 20 nt, synthetic construct
  source 1..20: mol_type = other RNA
ctcagtagccacaggccccg

SEQ ID NO: 23048 - RNA, 20 nt, synthetic construct
  source 1..20: mol_type = other RNA
tcagtagccacaggccccgt

SEQ ID NO: 23049 - RNA, 20 nt, synthetic construct
  source 1..20: mol_type = other RNA
cagtagccacaggccccgtg

SEQ ID NO: 23050 - RNA, 20 nt, synthetic construct
  source 1..20: mol_type = other RNA
cacggggcctgtggctactg

SEQ ID NO: 23051 - RNA, 20 nt, synthetic construct
  source 1..20: mol_type = other RNA
ctggggccccacggggcctg

SEQ ID NO: 23052 - RNA, 20 nt, synthetic construct
  source 1..20: mol_type = other RNA
atgacttctggggccccacg

SEQ ID NO: 23053 - RNA, 20 nt, synthetic construct
  source 1..20: mol_type = other RNA
gatgacttctggggccccac

SEQ ID NO: 23054 - RNA, 20 nt, synthetic construct
  source 1..20: mol_type = other RNA
cgatgacttctggggcccca

SEQ ID NO: 23055 - RNA, 20 nt, synthetic construct
  source 1..20: mol_type = other RNA
gggactgacgatgacttctg

SEQ ID NO: 23056 - RNA, 20 nt, synthetic construct
  source 1..20: mol_type = other RNA
aagtcatcgtcagtccccaa

SEQ ID NO: 23057 - RNA, 20 nt, synthetic construct
  source 1..20: mol_type = other RNA
tggggactgacgatgacttc

SEQ ID NO: 23058 - RNA, 20 nt, synthetic construct
  source 1..20: mol_type = other RNA
tccccaaaggcttcgtatgc

SEQ ID NO: 23059 - RNA, 20 nt, synthetic construct
  source 1..20: mol_type = other RNA
acctgcatacgaagcctttg

SEQ ID NO: 23060 - RNA, 20 nt, synthetic construct
  source 1..20: mol_type = other RNA
gacctgcatacgaagccttt

SEQ ID NO: 23061 - RNA, 20 nt, synthetic construct
  source 1..20: mol_type = other RNA
ggacctgcatacgaagcctt

SEQ ID NO: 23062 - RNA, 20 nt, synthetic construct
  source 1..20: mol_type = other RNA
cgtatgcaggtccccttgag

SEQ ID NO: 23063 - RNA, 20 nt, synthetic construct
  source 1..20: mol_type = other RNA
tgcaggtccccttgagaggc

SEQ ID NO: 23064 - RNA, 20 nt, synthetic construct
  source 1..20: mol_type = other RNA
tccccttgagaggcaggaga

SEQ ID NO: 23065 - RNA, 20 nt, synthetic construct
  source 1..20: mol_type = other RNA
gccttctcctgcctctcaag

SEQ ID NO: 23066 - RNA, 20 nt, synthetic construct
  source 1..20: mol_type = other RNA
tgccttctcctgcctctcaa

SEQ ID NO: 23067 - RNA, 20 nt, synthetic construct
  source 1..20: mol_type = other RNA
gtgccttctcctgcctctca

SEQ ID NO: 23068 - RNA, 20 nt, synthetic construct
  source 1..20: mol_type = other RNA
ggcacgcacaagagttccac

SEQ ID NO: 23069 - RNA, 20 nt, synthetic construct
  source 1..20: mol_type = other RNA
agttccaccggtactacctc

SEQ ID NO: 23070 - RNA, 20 nt, synthetic construct
  source 1..20: mol_type = other RNA
gttccaccggtactacctct

SEQ ID NO: 23071 - RNA, 20 nt, synthetic construct
  source 1..20: mol_type = other RNA
ttccaccggtactacctctg

SEQ ID NO: 23072 - RNA, 20 nt, synthetic construct
  source 1..20: mol_type = other RNA
ctccccagaggtagtaccgg

SEQ ID NO: 23073 - RNA, 20 nt, synthetic construct
  source 1..20: mol_type = other RNA
aagctccccagaggtagtac

SEQ ID NO: 23074 - RNA, 20 nt, synthetic construct
  source 1..20: mol_type = other RNA
ttcagaggaaagctccccag

SEQ ID NO: 23075 - RNA, 20 nt, synthetic construct
  source 1..20: mol_type = other RNA
agctttcctctgaaacagca

SEQ ID NO: 23076 - RNA, 20 nt, synthetic construct
  source 1..20: mol_type = other RNA
cctctgaaacagcaaggcag

SEQ ID NO: 23077 - RNA, 20 nt, synthetic construct
  source 1..20: mol_type = other RNA
ccgctgccttgctgtttcag

SEQ ID NO: 23078 - RNA, 20 nt, synthetic construct
  source 1..20: mol_type = other RNA
cagctccagattctcccgcc

SEQ ID NO: 23079 - RNA, 20 nt, synthetic construct
  source 1..20: mol_type = other RNA
ggaggccaggcgggagaatc

SEQ ID NO: 23080 - RNA, 20 nt, synthetic construct
  source 1..20: mol_type = other RNA
ggggctaggggaggccaggc

SEQ ID NO: 23081 - RNA, 20 nt, synthetic construct
  source 1..20: mol_type = other RNA
aggggctaggggaggccagg

SEQ ID NO: 23082 - RNA, 20 nt, synthetic construct
  source 1..20: mol_type = other RNA
cataggggctaggggaggcc

SEQ ID NO: 23083 - RNA, 20 nt, synthetic construct
  source 1..20: mol_type = other RNA
gcagccataggggctagggg

SEQ ID NO: 23084 - RNA, 20 nt, synthetic construct
  source 1..20: mol_type = other RNA
agtgcagccataggggctag

SEQ ID NO: 23085 - RNA, 20 nt, synthetic construct
  source 1..20: mol_type = other RNA
gcccctatggctgcactgta

SEQ ID NO: 23086 - RNA, 20 nt, synthetic construct
  source 1..20: mol_type = other RNA
acagtgcagccataggggct

SEQ ID NO: 23087 - RNA, 20 nt, synthetic construct
  source 1..20: mol_type = other RNA
ccctatggctgcactgtaag

SEQ ID NO: 23088 - RNA, 20 nt, synthetic construct
  source 1..20: mol_type = other RNA
cccttacagtgcagccatag

SEQ ID NO: 23089 - RNA, 20 nt, synthetic construct
  source 1..20: mol_type = other RNA
ccccttacagtgcagccata

SEQ ID NO: 23090 - RNA, 20 nt, synthetic construct
  source 1..20: mol_type = other RNA
gccccttacagtgcagccat

SEQ ID NO: 23091 - RNA, 20 nt, synthetic construct
  source 1..20: mol_type = other RNA
actgtaaggggcccttccca

SEQ ID NO: 23092 - RNA, 20 nt, synthetic construct
  source 1..20: mol_type = other RNA
taaggggcccttcccaaggc

SEQ ID NO: 23093 - RNA, 20 nt, synthetic construct
  source 1..20: mol_type = other RNA
cttcccaaggctggcctgcc

SEQ ID NO: 23094 - RNA, 20 nt, synthetic construct
  source 1..20: mol_type = other RNA
aggcaggccagccttgggaa

SEQ ID NO: 23095 - RNA, 20 nt, synthetic construct
  source 1..20: mol_type = other RNA
caggcaggccagccttggga

SEQ ID NO: 23096 - RNA, 20 nt, synthetic construct
  source 1..20: mol_type = other RNA
aggctggcctgcctggacca

SEQ ID NO: 23097 - RNA, 20 nt, synthetic construct
  source 1..20: mol_type = other RNA
ggtccaggcaggccagcctt

SEQ ID NO: 23098 - RNA, 20 nt, synthetic construct
  source 1..20: mol_type = other RNA
tggtccaggcaggccagcct

SEQ ID NO: 23099 - RNA, 20 nt, synthetic construct
  source 1..20: mol_type = other RNA
tggcctgcctggaccatggc

SEQ ID NO: 23100 - RNA, 20 nt, synthetic construct
  source 1..20: mol_type = other RNA
ggcctgcctggaccatggca

SEQ ID NO: 23101 - RNA, 20 nt, synthetic construct
  source 1..20: mol_type = other RNA
ctccctgccatggtccaggc

SEQ ID NO: 23102 - RNA, 20 nt, synthetic construct
  source 1..20: mol_type = other RNA
cacactccctgccatggtcc

SEQ ID NO: 23103 - RNA, 20 nt, synthetic construct
  source 1..20: mol_type = other RNA
atgggcggaggctgggctgg

SEQ ID NO: 23104 - RNA, 20 nt, synthetic construct
  source 1..20: mol_type = other RNA
gagatgggcggaggctgggc

SEQ ID NO: 23105 - RNA, 20 nt, synthetic construct
  source 1..20: mol_type = other RNA
aggggagatgggcggaggct

SEQ ID NO: 23106 - RNA, 20 nt, synthetic construct
  source 1..20: mol_type = other RNA
aaggggagatgggcggaggc

SEQ ID NO: 23107 - RNA, 20 nt, synthetic construct
  source 1..20: mol_type = other RNA
ggggaaggggagatgggcgg

SEQ ID NO: 23108 - RNA, 20 nt, synthetic construct
  source 1..20: mol_type = other RNA
agtggggaaggggagatggg

SEQ ID NO: 23109 - RNA, 20 nt, synthetic construct
  source 1..20: mol_type = other RNA
tccagtggggaaggggagat

SEQ ID NO: 23110 - RNA, 20 nt, synthetic construct
  source 1..20: mol_type = other RNA
ttccagtggggaaggggaga

SEQ ID NO: 23111 - RNA, 20 nt, synthetic construct
  source 1..20: mol_type = other RNA
cttctattccagtggggaag

SEQ ID NO: 23112 - RNA, 20 nt, synthetic construct
  source 1..20: mol_type = other RNA
acttctattccagtggggaa

SEQ ID NO: 23113 - RNA, 20 nt, synthetic construct
  source 1..20: mol_type = other RNA
cacttctattccagtgggga

SEQ ID NO: 23114 - RNA, 20 nt, synthetic construct
  source 1..20: mol_type = other RNA
gtggcacttctattccagtg

SEQ ID NO: 23115 - RNA, 20 nt, synthetic construct
  source 1..20: mol_type = other RNA
agtggcacttctattccagt

SEQ ID NO: 23116 - RNA, 20 nt, synthetic construct
  source 1..20: mol_type = other RNA
gagtggcacttctattccag

SEQ ID NO: 23117 - RNA, 20 nt, synthetic construct
  source 1..20: mol_type = other RNA
ccactctccccagcatgccc

SEQ ID NO: 23118 - RNA, 20 nt, synthetic construct
  source 1..20: mol_type = other RNA
ctctccccagcatgcccagg

SEQ ID NO: 23119 - RNA, 20 nt, synthetic construct
  source 1..20: mol_type = other RNA
tctccccagcatgcccaggt

SEQ ID NO: 23120 - RNA, 20 nt, synthetic construct
  source 1..20: mol_type = other RNA
cctgggcatgctggggagag

SEQ ID NO: 23121 - RNA, 20 nt, synthetic construct
  source 1..20: mol_type = other RNA
cccagcatgcccaggtgggc

SEQ ID NO: 23122 - RNA, 20 nt, synthetic construct
  source 1..20: mol_type = other RNA
ctgcccacctgggcatgctg

SEQ ID NO: 23123 - RNA, 20 nt, synthetic construct
  source 1..20: mol_type = other RNA
cctgcccacctgggcatgct

SEQ ID NO: 23124 - RNA, 20 nt, synthetic construct
  source 1..20: mol_type = other RNA
acctgcccacctgggcatgc

SEQ ID NO: 23125 - RNA, 20 nt, synthetic construct
  source 1..20: mol_type = other RNA
ctctctcaacctgcccacct

SEQ ID NO: 23126 - RNA, 20 nt, synthetic construct
  source 1..20: mol_type = other RNA
tctctctcaacctgcccacc

SEQ ID NO: 23127 - RNA, 20 nt, synthetic construct
  source 1..20: mol_type = other RNA
gggcaggttgagagagaaca

SEQ ID NO: 23128 - RNA, 20 nt, synthetic construct
  source 1..20: mol_type = other RNA
aacatggttcaaaagatgaa

SEQ ID NO: 23129 - RNA, 20 nt, synthetic construct
  source 1..20: mol_type = other RNA
acatggttcaaaagatgaaa

SEQ ID NO: 23130 - RNA, 20 nt, synthetic construct
  source 1..20: mol_type = other RNA
catggttcaaaagatgaaag

SEQ ID NO: 23131 - RNA, 20 nt, synthetic construct
  source 1..20: mol_type = other RNA
ttcaaaagatgaaaggggcc

SEQ ID NO: 23132 - RNA, 20 nt, synthetic construct
  source 1..20: mol_type = other RNA
atgaaaggggccaggcaccg

SEQ ID NO: 23133 - RNA, 20 nt, synthetic construct
  source 1..20: mol_type = other RNA
caggcaagagccacggtgcc

SEQ ID NO: 23134 - RNA, 20 nt, synthetic construct
  source 1..20: mol_type = other RNA
gagattgcaggcaagagcca

SEQ ID NO: 23135 - RNA, 20 nt, synthetic construct
  source 1..20: mol_type = other RNA
ttgcctgcaatctcagcaat

SEQ ID NO: 23136 - RNA, 20 nt, synthetic construct
  source 1..20: mol_type = other RNA
tgcctgcaatctcagcaatt

SEQ ID NO: 23137 - RNA, 20 nt, synthetic construct
  source 1..20: mol_type = other RNA
ttcccaattgctgagattgc

SEQ ID NO: 23138 - RNA, 20 nt, synthetic construct
  source 1..20: mol_type = other RNA
ggaagatcttgctcacgtcc

SEQ ID NO: 23139 - RNA, 20 nt, synthetic construct
  source 1..20: mol_type = other RNA
tcaggctaatctcaaactcc

SEQ ID NO: 23140 - RNA, 20 nt, synthetic construct
  source 1..20: mol_type = other RNA
tgagattagcctgagcaaca

SEQ ID NO: 23141 - RNA, 20 nt, synthetic construct
  source 1..20: mol_type = other RNA
gagattagcctgagcaacat

SEQ ID NO: 23142 - RNA, 20 nt, synthetic construct
  source 1..20: mol_type = other RNA
ggcggcttcccatgttgctc

SEQ ID NO: 23143 - RNA, 20 nt, synthetic construct
  source 1..20: mol_type = other RNA
tcttttttctgtagagaggg

SEQ ID NO: 23144 - RNA, 20 nt, synthetic construct
  source 1..20: mol_type = other RNA
ttttcttttttctgtagaga

SEQ ID NO: 23145 - RNA, 20 nt, synthetic construct
  source 1..20: mol_type = other RNA
tttttcttttttctgtagag

SEQ ID NO: 23146 - RNA, 20 nt, synthetic construct
  source 1..20: mol_type = other RNA
aaaaaagaaaaatatcagcc

SEQ ID NO: 23147 - RNA, 20 nt, synthetic construct
  source 1..20: mol_type = other RNA
agaaaaatatcagccaggca

SEQ ID NO: 23148 - RNA, 20 nt, synthetic construct
  source 1..20: mol_type = other RNA
aaaatatcagccaggcatgg

SEQ ID NO: 23149 - RNA, 20 nt, synthetic construct
  source 1..20: mol_type = other RNA
cagatgctcaccaccatgcc

SEQ ID NO: 23150 - RNA, 20 nt, synthetic construct
  source 1..20: mol_type = other RNA
ctgcagtcccagttctactc

SEQ ID NO: 23151 - RNA, 20 nt, synthetic construct
  source 1..20: mol_type = other RNA
cagtcccagttctactcagg

SEQ ID NO: 23152 - RNA, 20 nt, synthetic construct
  source 1..20: mol_type = other RNA
tcccagttctactcaggagg

SEQ ID NO: 23153 - RNA, 20 nt, synthetic construct
  source 1..20: mol_type = other RNA
cagttctactcaggaggcgg

SEQ ID NO: 23154 - RNA, 20 nt, synthetic construct
  source 1..20: mol_type = other RNA
tccgcctcctgagtagaact

SEQ ID NO: 23155 - RNA, 20 nt, synthetic construct
  source 1..20: mol_type = other RNA
ctccgcctcctgagtagaac

SEQ ID NO: 23156 - RNA, 20 nt, synthetic construct
  source 1..20: mol_type = other RNA
actcaggaggcggaggtggg

SEQ ID NO: 23157 - RNA, 20 nt, synthetic construct
  source 1..20: mol_type = other RNA
gaggattgtttgagctcaga

SEQ ID NO: 23158 - RNA, 20 nt, synthetic construct
  source 1..20: mol_type = other RNA
tgtttgagctcagaaggttt

SEQ ID NO: 23159 - RNA, 20 nt, synthetic construct
  source 1..20: mol_type = other RNA
ggcaggtttcctacccaaga

SEQ ID NO: 23160 - RNA, 20 nt, synthetic construct
  source 1..20: mol_type = other RNA
gggcaggtttcctacccaag

SEQ ID NO: 23161 - RNA, 20 nt, synthetic construct
  source 1..20: mol_type = other RNA
aacctgccccgtcccacatc

SEQ ID NO: 23162 - RNA, 20 nt, synthetic construct
  source 1..20: mol_type = other RNA
acctgccccgtcccacatca

SEQ ID NO: 23163 - RNA, 20 nt, synthetic construct
  source 1..20: mol_type = other RNA
cctgccccgtcccacatcag

SEQ ID NO: 23164 - RNA, 20 nt, synthetic construct
  source 1..20: mol_type = other RNA
cccctgatgtgggacggggc

SEQ ID NO: 23165 - RNA, 20 nt, synthetic construct
  source 1..20: mol_type = other RNA
ccgtcccacatcaggggcag

SEQ ID NO: 23166 - RNA, 20 nt, synthetic construct
  source 1..20: mol_type = other RNA
cgtcccacatcaggggcaga

SEQ ID NO: 23167 - RNA, 20 nt, synthetic construct
  source 1..20: mol_type = other RNA
tctgcccctgatgtgggacg

SEQ ID NO: 23168 - RNA, 20 nt, synthetic construct
  source 1..20: mol_type = other RNA
ctctgcccctgatgtgggac

SEQ ID NO: 23169 - RNA, 20 nt, synthetic construct
  source 1..20: mol_type = other RNA
cctctgcccctgatgtggga

SEQ ID NO: 23170 - RNA, 20 nt, synthetic construct
  source 1..20: mol_type = other RNA
catcaggggcagagggatgg

SEQ ID NO: 23171 - RNA, 20 nt, synthetic construct
  source 1..20: mol_type = other RNA
catccctctgcccctgatgt

SEQ ID NO: 23172 - RNA, 20 nt, synthetic construct
  source 1..20: mol_type = other RNA
ccatccctctgcccctgatg

SEQ ID NO: 23173 - RNA, 20 nt, synthetic construct
  source 1..20: mol_type = other RNA
tgggggaggtcagctgtggg

SEQ ID NO: 23174 - RNA, 20 nt, synthetic construct
  source 1..20: mol_type = other RNA
ggttgggggaggtcagctgt

SEQ ID NO: 23175 - RNA, 20 nt, synthetic construct
  source 1..20: mol_type = other RNA
gggttgggggaggtcagctg

SEQ ID NO: 23176 - RNA, 20 nt, synthetic construct
  source 1..20: mol_type = other RNA
atcgtgacaggggttggggg

SEQ ID NO: 23177 - RNA, 20 nt, synthetic construct
  source 1..20: mol_type = other RNA
agcatcgtgacaggggttgg

SEQ ID NO: 23178 - RNA, 20 nt, synthetic construct
  source 1..20: mol_type = other RNA
gagcatcgtgacaggggttg

SEQ ID NO: 23179 - RNA, 20 nt, synthetic construct
  source 1..20: mol_type = other RNA
ggagcatcgtgacaggggtt

SEQ ID NO: 23180 - RNA, 20 nt, synthetic construct
  source 1..20: mol_type = other RNA
gggagcatcgtgacaggggt

SEQ ID NO: 23181 - RNA, 20 nt, synthetic construct
  source 1..20: mol_type = other RNA
ggctgggagcatcgtgacag

SEQ ID NO: 23182 - RNA, 20 nt, synthetic construct
  source 1..20: mol_type = other RNA
aggctgggagcatcgtgaca

SEQ ID NO: 23183 - RNA, 20 nt, synthetic construct
  source 1..20: mol_type = other RNA
aaggctgggagcatcgtgac

SEQ ID NO: 23184 - RNA, 20 nt, synthetic construct
  source 1..20: mol_type = other RNA
tagtttgaaggggcaaggct

SEQ ID NO: 23185 - RNA, 20 nt, synthetic construct
  source 1..20: mol_type = other RNA
gtagtttgaaggggcaaggc

SEQ ID NO: 23186 - RNA, 20 nt, synthetic construct
  source 1..20: mol_type = other RNA
tcaggtagtttgaaggggca

SEQ ID NO: 23187 - RNA, 20 nt, synthetic construct
  source 1..20: mol_type = other RNA
tcggatcaggtagtttgaag

SEQ ID NO: 23188 - RNA, 20 nt, synthetic construct
  source 1..20: mol_type = other RNA
ctcggatcaggtagtttgaa

SEQ ID NO: 23189 - RNA, 20 nt, synthetic construct
  source 1..20: mol_type = other RNA
actcggatcaggtagtttga

SEQ ID NO: 23190 - RNA, 20 nt, synthetic construct
  source 1..20: mol_type = other RNA
aagcggcagagactcggatc

SEQ ID NO: 23191 - RNA, 20 nt, synthetic construct
  source 1..20: mol_type = other RNA
gagtctctgccgcttgagtg

SEQ ID NO: 23192 - RNA, 20 nt, synthetic construct
  source 1..20: mol_type = other RNA
tcactcaagcggcagagact

SEQ ID NO: 23193 - RNA, 20 nt, synthetic construct
  source 1..20: mol_type = other RNA
atagcacatcctcactcaag

SEQ ID NO: 23194 - RNA, 20 nt, synthetic construct
  source 1..20: mol_type = other RNA
tactcatctctcccgtatcc

SEQ ID NO: 23195 - RNA, 20 nt, synthetic construct
  source 1..20: mol_type = other RNA
cccgtatccaggccctcagt

SEQ ID NO: 23196 - RNA, 20 nt, synthetic construct
  source 1..20: mol_type = other RNA
ccgtatccaggccctcagta

SEQ ID NO: 23197 - RNA, 20 nt, synthetic construct
  source 1..20: mol_type = other RNA
cgtatccaggccctcagtag

SEQ ID NO: 23198 - RNA, 20 nt, synthetic construct
  source 1..20: mol_type = other RNA
cctactgagggcctggatac

SEQ ID NO: 23199 - RNA, 20 nt, synthetic construct
  source 1..20: mol_type = other RNA
ccctactgagggcctggata

SEQ ID NO: 23200 - RNA, 20 nt, synthetic construct
  source 1..20: mol_type = other RNA
gatgacccctactgagggcc

SEQ ID NO: 23201 - RNA, 20 nt, synthetic construct
  source 1..20: mol_type = other RNA
tcagtaggggtcatcacact

SEQ ID NO: 23202 - RNA, 20 nt, synthetic construct
  source 1..20: mol_type = other RNA
agtgtgatgacccctactga

SEQ ID NO: 23203 - RNA, 20 nt, synthetic construct
  source 1..20: mol_type = other RNA
aagtgtgatgacccctactg

SEQ ID NO: 23204 - RNA, 20 nt, synthetic construct
  source 1..20: mol_type = other RNA
ggtcatcacacttggtttcc

SEQ ID NO: 23205 - RNA, 20 nt, synthetic construct
  source 1..20: mol_type = other RNA
gaatgaacaattctttgtcc

SEQ ID NO: 23206 - RNA, 20 nt, synthetic construct
  source 1..20: mol_type = other RNA
gttcattctgcctaagatct

SEQ ID NO: 23207 - RNA, 20 nt, synthetic construct
  source 1..20: mol_type = other RNA
cattctgcctaagatcttgg

SEQ ID NO: 23208 - RNA, 20 nt, synthetic construct
  source 1..20: mol_type = other RNA
ctaagatcttggaggaagcg

SEQ ID NO: 23209 - RNA, 20 nt, synthetic construct
  source 1..20: mol_type = other RNA
taagatcttggaggaagcga

SEQ ID NO: 23210 - RNA, 20 nt, synthetic construct
  source 1..20: mol_type = other RNA
ctcgcttcctccaagatctt

SEQ ID NO: 23211 - RNA, 20 nt, synthetic construct
  source 1..20: mol_type = other RNA
tttttagtgggaatgtcatg

SEQ ID NO: 23212 - RNA, 20 nt, synthetic construct
  source 1..20: mol_type = other RNA
ctaaaaattcaactcctcct

SEQ ID NO: 23213 - RNA, 20 nt, synthetic construct
  source 1..20: mol_type = other RNA
ggaggagttgaatttttagt

SEQ ID NO: 23214 - RNA, 20 nt, synthetic construct
  source 1..20: mol_type = other RNA
aggaggagttgaatttttag

SEQ ID NO: 23215 - RNA, 20 nt, synthetic construct
  source 1..20: mol_type = other RNA
aattcaactcctcctcgggt

SEQ ID NO: 23216 - RNA, 20 nt, synthetic construct
  source 1..20: mol_type = other RNA
attcaactcctcctcgggtc

SEQ ID NO: 23217 - RNA, 20 nt, synthetic construct
  source 1..20: mol_type = other RNA
cctcctcgggtcgggtgcag

SEQ ID NO: 23218 - RNA, 20 nt, synthetic construct
  source 1..20: mol_type = other RNA
ccactgcacccgacccgagg

SEQ ID NO: 23219 - RNA, 20 nt, synthetic construct
  source 1..20: mol_type = other RNA
gagccactgcacccgacccg

SEQ ID NO: 23220 - RNA, 20 nt, synthetic construct
  source 1..20: mol_type = other RNA
gtggtgtctgggtttctccc

SEQ ID NO: 23221 - RNA, 20 nt, synthetic construct
  source 1..20: mol_type = other RNA
gtgagagacaaacacagcca

SEQ ID NO: 23222 - RNA, 20 nt, synthetic construct
  source 1..20: mol_type = other RNA
ggtgagagacaaacacagcc

SEQ ID NO: 23223 - RNA, 20 nt, synthetic construct
  source 1..20: mol_type = other RNA
tgtgtttgtctctcacccca

SEQ ID NO: 23224 - RNA, 20 nt, synthetic construct
  source 1..20: mol_type = other RNA
gagacagggaaagagccatg

SEQ ID NO: 23225 - RNA, 20 nt, synthetic construct
  source 1..20: mol_type = other RNA
ggagacagggaaagagccat

SEQ ID NO: 23226 - RNA, 20 nt, synthetic construct
  source 1..20: mol_type = other RNA
aggagacagggaaagagcca

SEQ ID NO: 23227 - RNA, 20 nt, synthetic construct
  source 1..20: mol_type = other RNA
ccctgtctcctgctcagccc

SEQ ID NO: 23228 - RNA, 20 nt, synthetic construct
  source 1..20: mol_type = other RNA
cctgtctcctgctcagccct

SEQ ID NO: 23229 - RNA, 20 nt, synthetic construct
  source 1..20: mol_type = other RNA
ccagggctgagcaggagaca

SEQ ID NO: 23230 - RNA, 20 nt, synthetic construct
  source 1..20: mol_type = other RNA
cccagggctgagcaggagac

SEQ ID NO: 23231 - RNA, 20 nt, synthetic construct
  source 1..20: mol_type = other RNA
tcctgctcagccctgggcct

SEQ ID NO: 23232 - RNA, 20 nt, synthetic construct
  source 1..20: mol_type = other RNA
acccaggcccagggctgagc

SEQ ID NO: 23233 - RNA, 20 nt, synthetic construct
  source 1..20: mol_type = other RNA
cctgggcctgggtcagccag

SEQ ID NO: 23234 - RNA, 20 nt, synthetic construct
  source 1..20: mol_type = other RNA
ctgggcctgggtcagccaga

SEQ ID NO: 23235 - RNA, 20 nt, synthetic construct
  source 1..20: mol_type = other RNA
ctctggctgacccaggccca

SEQ ID NO: 23236 - RNA, 20 nt, synthetic construct
  source 1..20: mol_type = other RNA
cctctggctgacccaggccc

SEQ ID NO: 23237 - RNA, 20 nt, synthetic construct
  source 1..20: mol_type = other RNA
gggtcagccagagggagttc

SEQ ID NO: 23238 - RNA, 20 nt, synthetic construct
  source 1..20: mol_type = other RNA
ggtcagccagagggagttct

SEQ ID NO: 23239 - RNA, 20 nt, synthetic construct
  source 1..20: mol_type = other RNA
gaactccctctggctgaccc

SEQ ID NO: 23240 - RNA, 20 nt, synthetic construct
  source 1..20: mol_type = other RNA
gggggacccagaactccctc

SEQ ID NO: 23241 - RNA, 20 nt, synthetic construct
  source 1..20: mol_type = other RNA
tcttcagcagacggtaaggg

SEQ ID NO: 23242 - RNA, 20 nt, synthetic construct
  source 1..20: mol_type = other RNA
atcttcagcagacggtaagg

SEQ ID NO: 23243 - RNA, 20 nt, synthetic construct
  source 1..20: mol_type = other RNA
catcttcagcagacggtaag

SEQ ID NO: 23244 - RNA, 20 nt, synthetic construct
  source 1..20: mol_type = other RNA
tcatcttcagcagacggtaa

SEQ ID NO: 23245 - RNA, 20 nt, synthetic construct
  source 1..20: mol_type = other RNA
ctcatcttcagcagacggta

SEQ ID NO: 23246 - RNA, 20 nt, synthetic construct
  source 1..20: mol_type = other RNA
ctgctgaagatgagcagctg

SEQ ID NO: 23247 - RNA, 20 nt, synthetic construct
  source 1..20: mol_type = other RNA
agctgctcatcttcagcaga

SEQ ID NO: 23248 - RNA, 20 nt, synthetic construct
  source 1..20: mol_type = other RNA
gctgaggtttctcctgctcc

SEQ ID NO: 23249 - RNA, 20 nt, synthetic construct
  source 1..20: mol_type = other RNA
ctgaggtttctcctgctcca

SEQ ID NO: 23250 - RNA, 20 nt, synthetic construct
  source 1..20: mol_type = other RNA
ggaactgagggccctggagc

SEQ ID NO: 23251 - RNA, 20 nt, synthetic construct
  source 1..20: mol_type = other RNA
gaggcaggaactgagggccc

SEQ ID NO: 23252 - RNA, 20 nt, synthetic construct
  source 1..20: mol_type = other RNA
tgagatgaggcaggaactga

SEQ ID NO: 23253 - RNA, 20 nt, synthetic construct
  source 1..20: mol_type = other RNA
atgagatgaggcaggaactg

SEQ ID NO: 23254 - RNA, 20 nt, synthetic construct
  source 1..20: mol_type = other RNA
tctgagtgatgagatgaggc

SEQ ID NO: 23255 - RNA, 20 nt, synthetic construct
  source 1..20: mol_type = other RNA
caactctgagtgatgagatg

SEQ ID NO: 23256 - RNA, 20 nt, synthetic construct
  source 1..20: mol_type = other RNA
ggtccagcctgaaagcacaa

SEQ ID NO: 23257 - RNA, 20 nt, synthetic construct
  source 1..20: mol_type = other RNA
gtccagcctgaaagcacaaa

SEQ ID NO: 23258 - RNA, 20 nt, synthetic construct
  source 1..20: mol_type = other RNA
cctgaaagcacaaagggagc

SEQ ID NO: 23259 - RNA, 20 nt, synthetic construct
  source 1..20: mol_type = other RNA
ctccctttgtgctttcaggc

SEQ ID NO: 23260 - RNA, 20 nt, synthetic construct
  source 1..20: mol_type = other RNA
ccggctccctttgtgctttc

SEQ ID NO: 23261 - RNA, 20 nt, synthetic construct
  source 1..20: mol_type = other RNA
caaagggagccgggtcctcc

SEQ ID NO: 23262 - RNA, 20 nt, synthetic construct
  source 1..20: mol_type = other RNA
aaagggagccgggtcctcct

SEQ ID NO: 23263 - RNA, 20 nt, synthetic construct
  source 1..20: mol_type = other RNA
tcctcctgggatcccccatg

SEQ ID NO: 23264 - RNA, 20 nt, synthetic construct
  source 1..20: mol_type = other RNA
accacatgggggatcccagg

SEQ ID NO: 23265 - RNA, 20 nt, synthetic construct
  source 1..20: mol_type = other RNA
ggatcccccatgtggtcccc

SEQ ID NO: 23266 - RNA, 20 nt, synthetic construct
  source 1..20: mol_type = other RNA
gggaccacatgggggatccc

SEQ ID NO: 23267 - RNA, 20 nt, synthetic construct
  source 1..20: mol_type = other RNA
catgtggtccccaggtcccc

SEQ ID NO: 23268 - RNA, 20 nt, synthetic construct
  source 1..20: mol_type = other RNA
gggacctggggaccacatgg

SEQ ID NO: 23269 - RNA, 20 nt, synthetic construct
  source 1..20: mol_type = other RNA
ggggacctggggaccacatg

SEQ ID NO: 23270 - RNA, 20 nt, synthetic construct
  source 1..20: mol_type = other RNA
tggggacctggggaccacat

SEQ ID NO: 23271 - RNA, 20 nt, synthetic construct
  source 1..20: mol_type = other RNA
ctggggacctggggaccaca

SEQ ID NO: 23272 - RNA, 20 nt, synthetic construct
  source 1..20: mol_type = other RNA
ttctgggccctggggacctg

SEQ ID NO: 23273 - RNA, 20 nt, synthetic construct
  source 1..20: mol_type = other RNA
gtccccagggcccagaatcc

SEQ ID NO: 23274 - RNA, 20 nt, synthetic construct
  source 1..20: mol_type = other RNA
tccccagggcccagaatcct

SEQ ID NO: 23275 - RNA, 20 nt, synthetic construct
  source 1..20: mol_type = other RNA
tcccaggattctgggccctg

SEQ ID NO: 23276 - RNA, 20 nt, synthetic construct
  source 1..20: mol_type = other RNA
gtcccaggattctgggccct

SEQ ID NO: 23277 - RNA, 20 nt, synthetic construct
  source 1..20: mol_type = other RNA
ggtcccaggattctgggccc

SEQ ID NO: 23278 - RNA, 20 nt, synthetic construct
  source 1..20: mol_type = other RNA
gtgacaggtcccaggattct

SEQ ID NO: 23279 - RNA, 20 nt, synthetic construct
  source 1..20: mol_type = other RNA
ggtgacaggtcccaggattc

SEQ ID NO: 23280 - RNA, 20 nt, synthetic construct
  source 1..20: mol_type = other RNA
ctgggacctgtcaccttctg

SEQ ID NO: 23281 - RNA, 20 nt, synthetic construct
  source 1..20: mol_type = other RNA
ctcagaaggtgacaggtccc

SEQ ID NO: 23282 - RNA, 20 nt, synthetic construct
  source 1..20: mol_type = other RNA
cctgtcaccttctgaggcag

SEQ ID NO: 23283 - RNA, 20 nt, synthetic construct
  source 1..20: mol_type = other RNA
ccgctgcctcagaaggtgac

SEQ ID NO: 23284 - RNA, 20 nt, synthetic construct
  source 1..20: mol_type = other RNA
ccttctgaggcagcggccgc

SEQ ID NO: 23285 - RNA, 20 nt, synthetic construct
  source 1..20: mol_type = other RNA
cttctgaggcagcggccgca

SEQ ID NO: 23286 - RNA, 20 nt, synthetic construct
  source 1..20: mol_type = other RNA
ctgaggcagcggccgcaggg

SEQ ID NO: 23287 - RNA, 20 nt, synthetic construct
  source 1..20: mol_type = other RNA
tgaggcagcggccgcagggt

SEQ ID NO: 23288 - RNA, 20 nt, synthetic construct
  source 1..20: mol_type = other RNA
cggccgcagggtgggttccc

SEQ ID NO: 23289 - RNA, 20 nt, synthetic construct
  source 1..20: mol_type = other RNA
ggtagagctggtaagaaact

SEQ ID NO: 23290 - RNA, 20 nt, synthetic construct
  source 1..20: mol_type = other RNA
gtagagctggtaagaaactt

SEQ ID NO: 23291 - RNA, 20 nt, synthetic construct
  source 1..20: mol_type = other RNA
agctggtaagaaacttgggt

SEQ ID NO: 23292 - RNA, 20 nt, synthetic construct
  source 1..20: mol_type = other RNA
atcggacaggggatggaaaa

SEQ ID NO: 23293 - RNA, 20 nt, synthetic construct
  source 1..20: mol_type = other RNA
ggggggtatcggacagggga

SEQ ID NO: 23294 - RNA, 20 nt, synthetic construct
  source 1..20: mol_type = other RNA
gttgggggggtatcggacag

SEQ ID NO: 23295 - RNA, 20 nt, synthetic construct
  source 1..20: mol_type = other RNA
ggttgggggggtatcggaca

SEQ ID NO: 23296 - RNA, 20 nt, synthetic construct
  source 1..20: mol_type = other RNA
gggttgggggggtatcggac

SEQ ID NO: 23297 - RNA, 20 nt, synthetic construct
  source 1..20: mol_type = other RNA
gaagagggttgggggggtat

SEQ ID NO: 23298 - RNA, 20 nt, synthetic construct
  source 1..20: mol_type = other RNA
cagagggaagagggttgggg

SEQ ID NO: 23299 - RNA, 20 nt, synthetic construct
  source 1..20: mol_type = other RNA
gcagagggaagagggttggg

SEQ ID NO: 23300 - RNA, 20 nt, synthetic construct
  source 1..20: mol_type = other RNA
ggcagagggaagagggttgg

SEQ ID NO: 23301 - RNA, 20 nt, synthetic construct
  source 1..20: mol_type = other RNA
gggcagagggaagagggttg

SEQ ID NO: 23302 - RNA, 20 nt, synthetic construct
  source 1..20: mol_type = other RNA
ccctcttccctctgcccaga

SEQ ID NO: 23303 - RNA, 20 nt, synthetic construct
  source 1..20: mol_type = other RNA
ctgggcagagggaagagggt

SEQ ID NO: 23304 - RNA, 20 nt, synthetic construct
  source 1..20: mol_type = other RNA
ccttctgggcagagggaaga

SEQ ID NO: 23305 - RNA, 20 nt, synthetic construct
  source 1..20: mol_type = other RNA
cccttctgggcagagggaag

SEQ ID NO: 23306 - RNA, 20 nt, synthetic construct
  source 1..20: mol_type = other RNA
tctgcccagaagggacccac

SEQ ID NO: 23307 - RNA, 20 nt, synthetic construct
  source 1..20: mol_type = other RNA
ctgcccagaagggacccaca

SEQ ID NO: 23308 - RNA, 20 nt, synthetic construct
  source 1..20: mol_type = other RNA
gtgggtcccttctgggcaga

SEQ ID NO: 23309 - RNA, 20 nt, synthetic construct
  source 1..20: mol_type = other RNA
tgtgggtcccttctgggcag

SEQ ID NO: 23310 - RNA, 20 nt, synthetic construct
  source 1..20: mol_type = other RNA
aggccctgtgggtcccttct

SEQ ID NO: 23311 - RNA, 20 nt, synthetic construct
  source 1..20: mol_type = other RNA
aaggccctgtgggtcccttc

SEQ ID NO: 23312 - RNA, 20 nt, synthetic construct
  source 1..20: mol_type = other RNA
gacccacagggccttacccc

SEQ ID NO: 23313 - RNA, 20 nt, synthetic construct
  source 1..20: mol_type = other RNA
cgcctggggtaaggccctgt

SEQ ID NO: 23314 - RNA, 20 nt, synthetic construct
  source 1..20: mol_type = other RNA
acgcctggggtaaggccctg

SEQ ID NO: 23315 - RNA, 20 nt, synthetic construct
  source 1..20: mol_type = other RNA
aaactcatacgcctggggta

SEQ ID NO: 23316 - RNA, 20 nt, synthetic construct
  source 1..20: mol_type = other RNA
aggcgtatgagtttgcaggc

SEQ ID NO: 23317 - RNA, 20 nt, synthetic construct
  source 1..20: mol_type = other RNA
cctgcaaactcatacgcctg

SEQ ID NO: 23318 - RNA, 20 nt, synthetic construct
  source 1..20: mol_type = other RNA
gcctgcaaactcatacgcct

SEQ ID NO: 23319 - RNA, 20 nt, synthetic construct
  source 1..20: mol_type = other RNA
tgcctgcaaactcatacgcc

SEQ ID NO: 23320 - RNA, 20 nt, synthetic construct
  source 1..20: mol_type = other RNA
gactgctctgtgaggggctc

SEQ ID NO: 23321 - RNA, 20 nt, synthetic construct
  source 1..20: mol_type = other RNA
gcgtgcgactgctctgtgag

SEQ ID NO: 23322 - RNA, 20 nt, synthetic construct
  source 1..20: mol_type = other RNA
ggcgtgcgactgctctgtga

SEQ ID NO: 23323 - RNA, 20 nt, synthetic construct
  source 1..20: mol_type = other RNA
tggcgtgcgactgctctgtg

SEQ ID NO: 23324 - RNA, 20 nt, synthetic construct
  source 1..20: mol_type = other RNA
gtcgcacgccaacgtcatcc

SEQ ID NO: 23325 - RNA, 20 nt, synthetic construct
  source 1..20: mol_type = other RNA
cagaacaacctggatgacgt

SEQ ID NO: 23326 - RNA, 20 nt, synthetic construct
  source 1..20: mol_type = other RNA
catccaggttgttctgctgc

SEQ ID NO: 23327 - RNA, 20 nt, synthetic construct
  source 1..20: mol_type = other RNA
agacctgcagcagaacaacc

SEQ ID NO: 23328 - RNA, 20 nt, synthetic construct
  source 1..20: mol_type = other RNA
gctgcaggtctagctccttc

SEQ ID NO: 23329 - RNA, 20 nt, synthetic construct
  source 1..20: mol_type = other RNA
caggtctagctccttcaggc

SEQ ID NO: 23330 - RNA, 20 nt, synthetic construct
  source 1..20: mol_type = other RNA
aggtctagctccttcaggct

SEQ ID NO: 23331 - RNA, 20 nt, synthetic construct
  source 1..20: mol_type = other RNA
ggtctagctccttcaggctg

SEQ ID NO: 23332 - RNA, 20 nt, synthetic construct
  source 1..20: mol_type = other RNA
tagctccttcaggctggggc

SEQ ID NO: 23333 - RNA, 20 nt, synthetic construct
  source 1..20: mol_type = other RNA
tagtgccagccccagcctga

SEQ ID NO: 23334 - RNA, 20 nt, synthetic construct
  source 1..20: mol_type = other RNA
ggggctggcactaagcacag

SEQ ID NO: 23335 - RNA, 20 nt, synthetic construct
  source 1..20: mol_type = other RNA
tggcactaagcacagaggcc

SEQ ID NO: 23336 - RNA, 20 nt, synthetic construct
  source 1..20: mol_type = other RNA
taagcacagaggccaggtcc

SEQ ID NO: 23337 - RNA, 20 nt, synthetic construct
  source 1..20: mol_type = other RNA
gtctgactgctgccaggacc

SEQ ID NO: 23338 - RNA, 20 nt, synthetic construct
  source 1..20: mol_type = other RNA
cctggcagcagtcagacgtg

SEQ ID NO: 23339 - RNA, 20 nt, synthetic construct
  source 1..20: mol_type = other RNA
cctcacgtctgactgctgcc

SEQ ID NO: 23340 - RNA, 20 nt, synthetic construct
  source 1..20: mol_type = other RNA
gccacagctgaccagcctgc

SEQ ID NO: 23341 - RNA, 20 nt, synthetic construct
  source 1..20: mol_type = other RNA
tcctgcaggctggtcagctg

SEQ ID NO: 23342 - RNA, 20 nt, synthetic construct
  source 1..20: mol_type = other RNA
cgtgtatctttcctgcaggc

SEQ ID NO: 23343 - RNA, 20 nt, synthetic construct
  source 1..20: mol_type = other RNA
ctggcgtgtatctttcctgc

SEQ ID NO: 23344 - RNA, 20 nt, synthetic construct
  source 1..20: mol_type = other RNA
ggaaagatacacgccagccc

SEQ ID NO: 23345 - RNA, 20 nt, synthetic construct
  source 1..20: mol_type = other RNA
cagcccaggtcattgtccta

SEQ ID NO: 23346 - RNA, 20 nt, synthetic construct
  source 1..20: mol_type = other RNA
agcccaggtcattgtcctaa

SEQ ID NO: 23347 - RNA, 20 nt, synthetic construct
  source 1..20: mol_type = other RNA
cttaggacaatgacctgggc

SEQ ID NO: 23348 - RNA, 20 nt, synthetic construct
  source 1..20: mol_type = other RNA
agcccttaggacaatgacct

SEQ ID NO: 23349 - RNA, 20 nt, synthetic construct
  source 1..20: mol_type = other RNA
gagcccttaggacaatgacc

SEQ ID NO: 23350 - RNA, 20 nt, synthetic construct
  source 1..20: mol_type = other RNA
gtcctaagggctcgctcttc

SEQ ID NO: 23351 - RNA, 20 nt, synthetic construct
  source 1..20: mol_type = other RNA
tcctaagggctcgctcttca

SEQ ID NO: 23352 - RNA, 20 nt, synthetic construct
  source 1..20: mol_type = other RNA
accctgaagagcgagccctt

SEQ ID NO: 23353 - RNA, 20 nt, synthetic construct
  source 1..20: mol_type = other RNA
gctcgctcttcagggtaact

SEQ ID NO: 23354 - RNA, 20 nt, synthetic construct
  source 1..20: mol_type = other RNA
ctcgctcttcagggtaacta

SEQ ID NO: 23355 - RNA, 20 nt, synthetic construct
  source 1..20: mol_type = other RNA
atcttccttctcagcatctg

SEQ ID NO: 23356 - RNA, 20 nt, synthetic construct
  source 1..20: mol_type = other RNA
tcagcatctgtggccttttg

SEQ ID NO: 23357 - RNA, 20 nt, synthetic construct
  source 1..20: mol_type = other RNA
cagcatctgtggccttttga

SEQ ID NO: 23358 - RNA, 20 nt, synthetic construct
  source 1..20: mol_type = other RNA
tctgtggccttttgagggtc

SEQ ID NO: 23359 - RNA, 20 nt, synthetic construct
  source 1..20: mol_type = other RNA
ctgtggccttttgagggtct

SEQ ID NO: 23360 - RNA, 20 nt, synthetic construct
  source 1..20: mol_type = other RNA
tgtcatcccagaccctcaaa

SEQ ID NO: 23361 - RNA, 20 nt, synthetic construct
  source 1..20: mol_type = other RNA
tgggagtgggaggagcctac

SEQ ID NO: 23362 - RNA, 20 nt, synthetic construct
  source 1..20: mol_type = other RNA
tcctcccactcccacaaagc

SEQ ID NO: 23363 - RNA, 20 nt, synthetic construct
  source 1..20: mol_type = other RNA
acctgctttgtgggagtggg

SEQ ID NO: 23364 - RNA, 20 nt, synthetic construct
  source 1..20: mol_type = other RNA
gagacctgctttgtgggagt

SEQ ID NO: 23365 - RNA, 20 nt, synthetic construct
  source 1..20: mol_type = other RNA
tgagacctgctttgtgggag

SEQ ID NO: 23366 - RNA, 20 nt, synthetic construct
  source 1..20: mol_type = other RNA
gaaggtgagacctgctttgt

SEQ ID NO: 23367 - RNA, 20 nt, synthetic construct
  source 1..20: mol_type = other RNA
agaaggtgagacctgctttg

SEQ ID NO: 23368 - RNA, 20 nt, synthetic construct
  source 1..20: mol_type = other RNA
agagggtaagagcagagaga

SEQ ID NO: 23369 - RNA, 20 nt, synthetic construct
  source 1..20: mol_type = other RNA
cttaccctctgcctgcctca

SEQ ID NO: 23370 - RNA, 20 nt, synthetic construct
  source 1..20: mol_type = other RNA
accctctgcctgcctcatgg

SEQ ID NO: 23371 - RNA, 20 nt, synthetic construct
  source 1..20: mol_type = other RNA
tctgcctgcctcatggtggc

SEQ ID NO: 23372 - RNA, 20 nt, synthetic construct
  source 1..20: mol_type = other RNA
gccaccatgaggcaggcaga

SEQ ID NO: 23373 - RNA, 20 nt, synthetic construct
  source 1..20: mol_type = other RNA
tgccaccatgaggcaggcag

SEQ ID NO: 23374 - RNA, 20 nt, synthetic construct
  source 1..20: mol_type = other RNA
actgcctgccaccatgaggc

SEQ ID NO: 23375 - RNA, 20 nt, synthetic construct
  source 1..20: mol_type = other RNA
gggaactgcctgccaccatg

SEQ ID NO: 23376 - RNA, 20 nt, synthetic construct
  source 1..20: mol_type = other RNA
ggtgggcagggggaggtgga

SEQ ID NO: 23377 - RNA, 20 nt, synthetic construct
  source 1..20: mol_type = other RNA
tggtgggcagggggaggtgg

SEQ ID NO: 23378 - RNA, 20 nt, synthetic construct
  source 1..20: mol_type = other RNA
tcttggtgggcagggggagg

SEQ ID NO: 23379 - RNA, 20 nt, synthetic construct
  source 1..20: mol_type = other RNA
tgttcttggtgggcaggggg

SEQ ID NO: 23380 - RNA, 20 nt, synthetic construct
  source 1..20: mol_type = other RNA
aattgttcttggtgggcagg

SEQ ID NO: 23381 - RNA, 20 nt, synthetic construct
  source 1..20: mol_type = other RNA
taattgttcttggtgggcag

SEQ ID NO: 23382 - RNA, 20 nt, synthetic construct
  source 1..20: mol_type = other RNA
gtaattgttcttggtgggca

SEQ ID NO: 23383 - RNA, 20 nt, synthetic construct
  source 1..20: mol_type = other RNA
agtaattgttcttggtgggc

SEQ ID NO: 23384 - RNA, 20 nt, synthetic construct
  source 1..20: mol_type = other RNA
ctgcagtaattgttcttggt

SEQ ID NO: 23385 - RNA, 20 nt, synthetic construct
  source 1..20: mol_type = other RNA
actgcagtaattgttcttgg

SEQ ID NO: 23386 - RNA, 20 nt, synthetic construct
  source 1..20: mol_type = other RNA
gcgactgcagtaattgttct

SEQ ID NO: 23387 - RNA, 20 nt, synthetic construct
  source 1..20: mol_type = other RNA
agtcgctgtagcttgcagct

SEQ ID NO: 23388 - RNA, 20 nt, synthetic construct
  source 1..20: mol_type = other RNA
agctcggctgtctcagtctc

SEQ ID NO: 23389 - RNA, 20 nt, synthetic construct
  source 1..20: mol_type = other RNA
gctgtctcagtctctggcaa

SEQ ID NO: 23390 - RNA, 20 nt, synthetic construct
  source 1..20: mol_type = other RNA
cagtctctggcaaaggtgtt

SEQ ID NO: 23391 - RNA, 20 nt, synthetic construct
  source 1..20: mol_type = other RNA
ttcaatgtgctcacggatgc

SEQ ID NO: 23392 - RNA, 20 nt, synthetic construct
  source 1..20: mol_type = other RNA
ccgtgagcacattgaagctc

SEQ ID NO: 23393 - RNA, 20 nt, synthetic construct
  source 1..20: mol_type = other RNA
cctgagcttcaatgtgctca

SEQ ID NO: 23394 - RNA, 20 nt, synthetic construct
  source 1..20: mol_type = other RNA
attgaagctcaggtccagct

SEQ ID NO: 23395 - RNA, 20 nt, synthetic construct
  source 1..20: mol_type = other RNA
agctcaggtccagctcggtc

SEQ ID NO: 23396 - RNA, 20 nt, synthetic construct
  source 1..20: mol_type = other RNA
gctcaggtccagctcggtca

SEQ ID NO: 23397 - RNA, 20 nt, synthetic construct
  source 1..20: mol_type = other RNA
ggtccagctcggtcagggtc

SEQ ID NO: 23398 - RNA, 20 nt, synthetic construct
  source 1..20: mol_type = other RNA
cagctcggtcagggtctggt

SEQ ID NO: 23399 - RNA, 20 nt, synthetic construct
  source 1..20: mol_type = other RNA
caaccagaccctgaccgagc

SEQ ID NO: 23400 - RNA, 20 nt, synthetic construct
  source 1..20: mol_type = other RNA
ctggttggctctcagcccaa

SEQ ID NO: 23401 - RNA, 20 nt, synthetic construct
  source 1..20: mol_type = other RNA
tggctctcagcccaaaggca

SEQ ID NO: 23402 - RNA, 20 nt, synthetic construct
  source 1..20: mol_type = other RNA
actgcaaggaccttgccttt

SEQ ID NO: 23403 - RNA, 20 nt, synthetic construct
  source 1..20: mol_type = other RNA
gactgcaaggaccttgcctt

SEQ ID NO: 23404 - RNA, 20 nt, synthetic construct
  source 1..20: mol_type = other RNA
ccttgcagtcctcagctgtg

SEQ ID NO: 23405 - RNA, 20 nt, synthetic construct
  source 1..20: mol_type = other RNA
cctcacagctgaggactgca

SEQ ID NO: 23406 - RNA, 20 nt, synthetic construct
  source 1..20: mol_type = other RNA
tggctgtggcctcacagctg

SEQ ID NO: 23407 - RNA, 20 nt, synthetic construct
  source 1..20: mol_type = other RNA
ggccacagccagccaacctg

SEQ ID NO: 23408 - RNA, 20 nt, synthetic construct
  source 1..20: mol_type = other RNA
ttccacaggttggctggctg

SEQ ID NO: 23409 - RNA, 20 nt, synthetic construct
  source 1..20: mol_type = other RNA
tgtgtcttccacaggttggc

SEQ ID NO: 23410 - RNA, 20 nt, synthetic construct
  source 1..20: mol_type = other RNA
ggtgtgtgtcttccacaggt

SEQ ID NO: 23411 - RNA, 20 nt, synthetic construct
  source 1..20: mol_type = other RNA
catgggtgtgtgtcttccac

SEQ ID NO: 23412 - RNA, 20 nt, synthetic construct
  source 1..20: mol_type = other RNA
gacacacacccatggtcttc

SEQ ID NO: 23413 - RNA, 20 nt, synthetic construct
  source 1..20: mol_type = other RNA
gtgagtaacctgaagaccat

SEQ ID NO: 23414 - RNA, 20 nt, synthetic construct
  source 1..20: mol_type = other RNA
ggtgagtaacctgaagacca

SEQ ID NO: 23415 - RNA, 20 nt, synthetic construct
  source 1..20: mol_type = other RNA
tgggtgtctgttgaatcaac

SEQ ID NO: 23416 - RNA, 20 nt, synthetic construct
  source 1..20: mol_type = other RNA
ggtgattaatggttgcttat

SEQ ID NO: 23417 - RNA, 20 nt, synthetic construct
  source 1..20: mol_type = other RNA
aggtgattaatggttgctta

SEQ ID NO: 23418 - RNA, 20 nt, synthetic construct
  source 1..20: mol_type = other RNA
ttaatcacctactatgcacc

SEQ ID NO: 23419 - RNA, 20 nt, synthetic construct
  source 1..20: mol_type = other RNA
ggtgcatagtaggtgattaa

SEQ ID NO: 23420 - RNA, 20 nt, synthetic construct
  source 1..20: mol_type = other RNA
cctactatgcaccaggcctg

SEQ ID NO: 23421 - RNA, 20 nt, synthetic construct
  source 1..20: mol_type = other RNA
ctactatgcaccaggcctgt

SEQ ID NO: 23422 - RNA, 20 nt, synthetic construct
  source 1..20: mol_type = other RNA
ccacaggcctggtgcatagt

SEQ ID NO: 23423 - RNA, 20 nt, synthetic construct
  source 1..20: mol_type = other RNA
atgcaccaggcctgtgggcc

SEQ ID NO: 23424 - RNA, 20 nt, synthetic construct
  source 1..20: mol_type = other RNA
caggcctgtgggccaggcag

SEQ ID NO: 23425 - RNA, 20 nt, synthetic construct
  source 1..20: mol_type = other RNA
ctctgcctggcccacaggcc

SEQ ID NO: 23426 - RNA, 20 nt, synthetic construct
  source 1..20: mol_type = other RNA
tagacctctgcctggcccac

SEQ ID NO: 23427 - RNA, 20 nt, synthetic construct
  source 1..20: mol_type = other RNA
cgttgaggccttctctggcc

SEQ ID NO: 23428 - RNA, 20 nt, synthetic construct
  source 1..20: mol_type = other RNA
tcgttgaggccttctctggc

SEQ ID NO: 23429 - RNA, 20 nt, synthetic construct
  source 1..20: mol_type = other RNA
atattcgttgaggccttctc

SEQ ID NO: 23430 - RNA, 20 nt, synthetic construct
  source 1..20: mol_type = other RNA
tatttatcaaatattcgttg

SEQ ID NO: 23431 - RNA, 20 nt, synthetic construct
  source 1..20: mol_type = other RNA
agaagctgagtctgggctga

SEQ ID NO: 23432 - RNA, 20 nt, synthetic construct
  source 1..20: mol_type = other RNA
cagaagctgagtctgggctg

SEQ ID NO: 23433 - RNA, 20 nt, synthetic construct
  source 1..20: mol_type = other RNA
cccagactcagcttctgcct

SEQ ID NO: 23434 - RNA, 20 nt, synthetic construct
  source 1..20: mol_type = other RNA
ccaaggcagaagctgagtct

SEQ ID NO: 23435 - RNA, 20 nt, synthetic construct
  source 1..20: mol_type = other RNA
tccaaggcagaagctgagtc

SEQ ID NO: 23436 - RNA, 20 nt, synthetic construct
  source 1..20: mol_type = other RNA
agggatggggaagagatcca

SEQ ID NO: 23437 - RNA, 20 nt, synthetic construct
  source 1..20: mol_type = other RNA
tctgttctgaagcagggatg

SEQ ID NO: 23438 - RNA, 20 nt, synthetic construct
  source 1..20: mol_type = other RNA
ttctgttctgaagcagggat

SEQ ID NO: 23439 - RNA, 20 nt, synthetic construct
  source 1..20: mol_type = other RNA
cctgcttcagaacagaaccc

SEQ ID NO: 23440 - RNA, 20 nt, synthetic construct
  source 1..20: mol_type = other RNA
ctgggttctgttctgaagca

SEQ ID NO: 23441 - RNA, 20 nt, synthetic construct
  source 1..20: mol_type = other RNA
cctgggttctgttctgaagc

SEQ ID NO: 23442 - RNA, 20 nt, synthetic construct
  source 1..20: mol_type = other RNA
acccaggccagactcaccgc

SEQ ID NO: 23443 - RNA, 20 nt, synthetic construct
  source 1..20: mol_type = other RNA
cccaggccagactcaccgca

SEQ ID NO: 23444 - RNA, 20 nt, synthetic construct
  source 1..20: mol_type = other RNA
ccctgcggtgagtctggcct

SEQ ID NO: 23445 - RNA, 20 nt, synthetic construct
  source 1..20: mol_type = other RNA
accctgcggtgagtctggcc

SEQ ID NO: 23446 - RNA, 20 nt, synthetic construct
  source 1..20: mol_type = other RNA
agactcaccgcagggtctcc

SEQ ID NO: 23447 - RNA, 20 nt, synthetic construct
  source 1..20: mol_type = other RNA
tggagaccctgcggtgagtc

SEQ ID NO: 23448 - RNA, 20 nt, synthetic construct
  source 1..20: mol_type = other RNA
agggtctccaggaggcagcg

SEQ ID NO: 23449 - RNA, 20 nt, synthetic construct
  source 1..20: mol_type = other RNA
gctgcctcctggagaccctg

SEQ ID NO: 23450 - RNA, 20 nt, synthetic construct
  source 1..20: mol_type = other RNA
ggaggcagcgagggcgtctc

SEQ ID NO: 23451 - RNA, 20 nt, synthetic construct
  source 1..20: mol_type = other RNA
gaggcagcgagggcgtctca

SEQ ID NO: 23452 - RNA, 20 nt, synthetic construct
  source 1..20: mol_type = other RNA
gagacgccctcgctgcctcc

SEQ ID NO: 23453 - RNA, 20 nt, synthetic construct
  source 1..20: mol_type = other RNA
aaagactcttcactgcagag

SEQ ID NO: 23454 - RNA, 20 nt, synthetic construct
  source 1..20: mol_type = other RNA
ggctcagcgagtttccactt

SEQ ID NO: 23455 - RNA, 20 nt, synthetic construct
  source 1..20: mol_type = other RNA
cacttaggtccagctccttc

SEQ ID NO: 23456 - RNA, 20 nt, synthetic construct
  source 1..20: mol_type = other RNA
ctgaaggagctggacctaag

SEQ ID NO: 23457 - RNA, 20 nt, synthetic construct
  source 1..20: mol_type = other RNA
gtccagctccttcaggtttc

SEQ ID NO: 23458 - RNA, 20 nt, synthetic construct
  source 1..20: mol_type = other RNA
caccagaaacctgaaggagc

SEQ ID NO: 23459 - RNA, 20 nt, synthetic construct
  source 1..20: mol_type = other RNA
tcaggtttctggtgaccttg

SEQ ID NO: 23460 - RNA, 20 nt, synthetic construct
  source 1..20: mol_type = other RNA
caaggtcaccagaaacctga

SEQ ID NO: 23461 - RNA, 20 nt, synthetic construct
  source 1..20: mol_type = other RNA
gtttctggtgaccttgagga

SEQ ID NO: 23462 - RNA, 20 nt, synthetic construct
  source 1..20: mol_type = other RNA
gattctcttctccgtcctca

SEQ ID NO: 23463 - RNA, 20 nt, synthetic construct
  source 1..20: mol_type = other RNA
ggagaagagaatctgccaat

SEQ ID NO: 23464 - RNA, 20 nt, synthetic construct
  source 1..20: mol_type = other RNA
tgccaataggcatctgtgac

SEQ ID NO: 23465 - RNA, 20 nt, synthetic construct
  source 1..20: mol_type = other RNA
gccaataggcatctgtgact

SEQ ID NO: 23466 - RNA, 20 nt, synthetic construct
  source 1..20: mol_type = other RNA
tcccagtcacagatgcctat

SEQ ID NO: 23467 - RNA, 20 nt, synthetic construct
  source 1..20: mol_type = other RNA
ctgggacccacctgaacctg

SEQ ID NO: 23468 - RNA, 20 nt, synthetic construct
  source 1..20: mol_type = other RNA
tgggacccacctgaacctga

SEQ ID NO: 23469 - RNA, 20 nt, synthetic construct
  source 1..20: mol_type = other RNA
gggacccacctgaacctgag

SEQ ID NO: 23470 - RNA, 20 nt, synthetic construct
  source 1..20: mol_type = other RNA
ggacccacctgaacctgagg

SEQ ID NO: 23471 - RNA, 20 nt, synthetic construct
  source 1..20: mol_type = other RNA
tctccccctcaggttcaggt

SEQ ID NO: 23472 - RNA, 20 nt, synthetic construct
  source 1..20: mol_type = other RNA
ctctccccctcaggttcagg

SEQ ID NO: 23473 - RNA, 20 nt, synthetic construct
  source 1..20: mol_type = other RNA
gaacctgagggggagagaga

SEQ ID NO: 23474 - RNA, 20 nt, synthetic construct
  source 1..20: mol_type = other RNA
tctctctccccctcaggttc

SEQ ID NO: 23475 - RNA, 20 nt, synthetic construct
  source 1..20: mol_type = other RNA
tgagggggagagagaaggac

SEQ ID NO: 23476 - RNA, 20 nt, synthetic construct
  source 1..20: mol_type = other RNA
tgtccttctctctccccctc

SEQ ID NO: 23477 - RNA, 20 nt, synthetic construct
  source 1..20: mol_type = other RNA
caggagagatgtgatgtgtc

SEQ ID NO: 23478 - RNA, 20 nt, synthetic construct
  source 1..20: mol_type = other RNA
agagatgtgatgtgtctggc

SEQ ID NO: 23479 - RNA, 20 nt, synthetic construct
  source 1..20: mol_type = other RNA
gagatgtgatgtgtctggca

SEQ ID NO: 23480 - RNA, 20 nt, synthetic construct
  source 1..20: mol_type = other RNA
agatgtgatgtgtctggcag

SEQ ID NO: 23481 - RNA, 20 nt, synthetic construct
  source 1..20: mol_type = other RNA
atgtgtctggcaggggtttg

SEQ ID NO: 23482 - RNA, 20 nt, synthetic construct
  source 1..20: mol_type = other RNA
ccagccctgcacaacacagt

SEQ ID NO: 23483 - RNA, 20 nt, synthetic construct
  source 1..20: mol_type = other RNA
cagccctgcacaacacagtt

SEQ ID NO: 23484 - RNA, 20 nt, synthetic construct
  source 1..20: mol_type = other RNA
caactgtgttgtgcagggct

SEQ ID NO: 23485 - RNA, 20 nt, synthetic construct
  source 1..20: mol_type = other RNA
ccaactgtgttgtgcagggc

SEQ ID NO: 23486 - RNA, 20 nt, synthetic construct
  source 1..20: mol_type = other RNA
aagcccaactgtgttgtgca

SEQ ID NO: 23487 - RNA, 20 nt, synthetic construct
  source 1..20: mol_type = other RNA
aaagcccaactgtgttgtgc

SEQ ID NO: 23488 - RNA, 20 nt, synthetic construct
  source 1..20: mol_type = other RNA
gctttgtccccctgagcacc

SEQ ID NO: 23489 - RNA, 20 nt, synthetic construct
  source 1..20: mol_type = other RNA
ccctgagcaccaggccacag

SEQ ID NO: 23490 - RNA, 20 nt, synthetic construct
  source 1..20: mol_type = other RNA
cctgagcaccaggccacagc

SEQ ID NO: 23491 - RNA, 20 nt, synthetic construct
  source 1..20: mol_type = other RNA
gctgtggcctggtgctcagg

SEQ ID NO: 23492 - RNA, 20 nt, synthetic construct
  source 1..20: mol_type = other RNA
cgctgtggcctggtgctcag

SEQ ID NO: 23493 - RNA, 20 nt, synthetic construct
  source 1..20: mol_type = other RNA
ccgctgtggcctggtgctca

SEQ ID NO: 23494 - RNA, 20 nt, synthetic construct
  source 1..20: mol_type = other RNA
cccgctgtggcctggtgctc

SEQ ID NO: 23495 - RNA, 20 nt, synthetic construct
  source 1..20: mol_type = other RNA
tgggggtggctaaaggatca

SEQ ID NO: 23496 - RNA, 20 nt, synthetic construct
  source 1..20: mol_type = other RNA
gtgggggtggctaaaggatc

SEQ ID NO: 23497 - RNA, 20 nt, synthetic construct
  source 1..20: mol_type = other RNA
cctttagccacccccacccc

SEQ ID NO: 23498 - RNA, 20 nt, synthetic construct
  source 1..20: mol_type = other RNA
agccacccccacccccggcc

SEQ ID NO: 23499 - RNA, 20 nt, synthetic construct
  source 1..20: mol_type = other RNA
agcctggccgggggtggggg

SEQ ID NO: 23500 - RNA, 20 nt, synthetic construct
  source 1..20: mol_type = other RNA
ctgagcctggccgggggtgg

SEQ ID NO: 23501 - RNA, 20 nt, synthetic construct
  source 1..20: mol_type = other RNA
actgagcctggccgggggtg

SEQ ID NO: 23502 - RNA, 20 nt, synthetic construct
  source 1..20: mol_type = other RNA
cactgagcctggccgggggt

SEQ ID NO: 23503 - RNA, 20 nt, synthetic construct
  source 1..20: mol_type = other RNA
tcactgagcctggccggggg

SEQ ID NO: 23504 - RNA, 20 nt, synthetic construct
  source 1..20: mol_type = other RNA
tgctcactgagcctggccgg

SEQ ID NO: 23505 - RNA, 20 nt, synthetic construct
  source 1..20: mol_type = other RNA
atgctcactgagcctggccg

SEQ ID NO: 23506 - RNA, 20 nt, synthetic construct
  source 1..20: mol_type = other RNA
catgctcactgagcctggcc

SEQ ID NO: 23507 - RNA, 20 nt, synthetic construct
  source 1..20: mol_type = other RNA
gcatgctcactgagcctggc

SEQ ID NO: 23508 - RNA, 20 nt, synthetic construct
  source 1..20: mol_type = other RNA
aggctcagtgagcatgcctc

SEQ ID NO: 23509 - RNA, 20 nt, synthetic construct
  source 1..20: mol_type = other RNA
agaggcatgctcactgagcc

SEQ ID NO: 23510 - RNA, 20 nt, synthetic construct
  source 1..20: mol_type = other RNA
tgagcatgcctctggtgctc

SEQ ID NO: 23511 - RNA, 20 nt, synthetic construct
  source 1..20: mol_type = other RNA
cctctggtgctcaggtcact

SEQ ID NO: 23512 - RNA, 20 nt, synthetic construct
  source 1..20: mol_type = other RNA
ctctggtgctcaggtcactc

SEQ ID NO: 23513 - RNA, 20 nt, synthetic construct
  source 1..20: mol_type = other RNA
ccgagtgacctgagcaccag

SEQ ID NO: 23514 - RNA, 20 nt, synthetic construct
  source 1..20: mol_type = other RNA
gctcaggtcactcgggctta

SEQ ID NO: 23515 - RNA, 20 nt, synthetic construct
  source 1..20: mol_type = other RNA
tcgggcttatggactgacag

SEQ ID NO: 23516 - RNA, 20 nt, synthetic construct
  source 1..20: mol_type = other RNA
tgacagaggagctgcagaca

SEQ ID NO: 23517 - RNA, 20 nt, synthetic construct
  source 1..20: mol_type = other RNA
gacagaggagctgcagacat

SEQ ID NO: 23518 - RNA, 20 nt, synthetic construct
  source 1..20: mol_type = other RNA
agaggagctgcagacatggg

SEQ ID NO: 23519 - RNA, 20 nt, synthetic construct
  source 1..20: mol_type = other RNA
agctgcagacatgggtggtt

SEQ ID NO: 23520 - RNA, 20 nt, synthetic construct
  source 1..20: mol_type = other RNA
gctgcagacatgggtggttt

SEQ ID NO: 23521 - RNA, 20 nt, synthetic construct
  source 1..20: mol_type = other RNA
tgggtggtttgggtactcac

SEQ ID NO: 23522 - RNA, 20 nt, synthetic construct
  source 1..20: mol_type = other RNA
gggtactcacaggactacca

SEQ ID NO: 23523 - RNA, 20 nt, synthetic construct
  source 1..20: mol_type = other RNA
tactcacaggactaccatgg

SEQ ID NO: 23524 - RNA, 20 nt, synthetic construct
  source 1..20: mol_type = other RNA
actcacaggactaccatggt

SEQ ID NO: 23525 - RNA, 20 nt, synthetic construct
  source 1..20: mol_type = other RNA
ctcacaggactaccatggtg

SEQ ID NO: 23526 - RNA, 20 nt, synthetic construct
  source 1..20: mol_type = other RNA
atcaacatggagccccacca

SEQ ID NO: 23527 - RNA, 20 nt, synthetic construct
  source 1..20: mol_type = other RNA
gcaggcagcacagatcaaca

SEQ ID NO: 23528 - RNA, 20 nt, synthetic construct
  source 1..20: mol_type = other RNA
agcttcagctgattgagggc

SEQ ID NO: 23529 - RNA, 20 nt, synthetic construct
  source 1..20: mol_type = other RNA
aagaagcttcagctgattga

SEQ ID NO: 23530 - RNA, 20 nt, synthetic construct
  source 1..20: mol_type = other RNA
gaagaagcttcagctgattg

SEQ ID NO: 23531 - RNA, 20 nt, synthetic construct
  source 1..20: mol_type = other RNA
tcagctgaagcttcttcacg

SEQ ID NO: 23532 - RNA, 20 nt, synthetic construct
  source 1..20: mol_type = other RNA
gctgaagcttcttcacgtgg

SEQ ID NO: 23533 - RNA, 20 nt, synthetic construct
  source 1..20: mol_type = other RNA
catgtgtgtagaaacagaca

SEQ ID NO: 23534 - RNA, 20 nt, synthetic construct
  source 1..20: mol_type = other RNA
acatgcccatttcttcgaaa

SEQ ID NO: 23535 - RNA, 20 nt, synthetic construct
  source 1..20: mol_type = other RNA
catgcccatttcttcgaaat

SEQ ID NO: 23536 - RNA, 20 nt, synthetic construct
  source 1..20: mol_type = other RNA
atggcccatttcgaagaaat

SEQ ID NO: 23537 - RNA, 20 nt, synthetic construct
  source 1..20: mol_type = other RNA
gatggcccatttcgaagaaa

SEQ ID NO: 23538 - RNA, 20 nt, synthetic construct
  source 1..20: mol_type = other RNA
aatgggccatcacttgtgtc

SEQ ID NO: 23539 - RNA, 20 nt, synthetic construct
  source 1..20: mol_type = other RNA
aacgttcctgacacaagtga

SEQ ID NO: 23540 - RNA, 20 nt, synthetic construct
  source 1..20: mol_type = other RNA
tccgagtctcgtacaagcag

SEQ ID NO: 23541 - RNA, 20 nt, synthetic construct
  source 1..20: mol_type = other RNA
gagtctcgtacaagcagtgg

SEQ ID NO: 23542 - RNA, 20 nt, synthetic construct
  source 1..20: mol_type = other RNA
agtctcgtacaagcagtgga

SEQ ID NO: 23543 - RNA, 20 nt, synthetic construct
  source 1..20: mol_type = other RNA
tccactgcttgtacgagact

SEQ ID NO: 23544 - RNA, 20 nt, synthetic construct
  source 1..20: mol_type = other RNA
tggagggactccagagagtg

SEQ ID NO: 23545 - RNA, 20 nt, synthetic construct
  source 1..20: mol_type = other RNA
gctgctgcagccacactctc

SEQ ID NO: 23546 - RNA, 20 nt, synthetic construct
  source 1..20: mol_type = other RNA
gtggctgcagcagcagctgc

SEQ ID NO: 23547 - RNA, 20 nt, synthetic construct
  source 1..20: mol_type = other RNA
tggctgcagcagcagctgca

SEQ ID NO: 23548 - RNA, 20 nt, synthetic construct
  source 1..20: mol_type = other RNA
tgcagcagcagctgcaggga

SEQ ID NO: 23549 - RNA, 20 nt, synthetic construct
  source 1..20: mol_type = other RNA
gcagcagcagctgcagggac

SEQ ID NO: 23550 - RNA, 20 nt, synthetic construct
  source 1..20: mol_type = other RNA
gggacgggacccactgcatc

SEQ ID NO: 23551 - RNA, 20 nt, synthetic construct
  source 1..20: mol_type = other RNA
ggggaggaacctgatgcagt

SEQ ID NO: 23552 - RNA, 20 nt, synthetic construct
  source 1..20: mol_type = other RNA
aggggaggaacctgatgcag

SEQ ID NO: 23553 - RNA, 20 nt, synthetic construct
  source 1..20: mol_type = other RNA
ggttcctcccctgagacagc

SEQ ID NO: 23554 - RNA, 20 nt, synthetic construct
  source 1..20: mol_type = other RNA
actgccggctgtctcagggg

SEQ ID NO: 23555 - RNA, 20 nt, synthetic construct
  source 1..20: mol_type = other RNA
ttcactgccggctgtctcag

SEQ ID NO: 23556 - RNA, 20 nt, synthetic construct
  source 1..20: mol_type = other RNA
tttcactgccggctgtctca

SEQ ID NO: 23557 - RNA, 20 nt, synthetic construct
  source 1..20: mol_type = other RNA
ctttcactgccggctgtctc

SEQ ID NO: 23558 - RNA, 20 nt, synthetic construct
  source 1..20: mol_type = other RNA
tggagaacatctttcactgc

SEQ ID NO: 23559 - RNA, 20 nt, synthetic construct
  source 1..20: mol_type = other RNA
tgatgagggggagagagaga

SEQ ID NO: 23560 - RNA, 20 nt, synthetic construct
  source 1..20: mol_type = other RNA
tctccccctcatcacttaac

SEQ ID NO: 23561 - RNA, 20 nt, synthetic construct
  source 1..20: mol_type = other RNA
gggcctgttaagtgatgagg

SEQ ID NO: 23562 - RNA, 20 nt, synthetic construct
  source 1..20: mol_type = other RNA
catcacttaacaggcccaat

SEQ ID NO: 23563 - RNA, 20 nt, synthetic construct
  source 1..20: mol_type = other RNA
ttgggcctgttaagtgatga

SEQ ID NO: 23564 - RNA, 20 nt, synthetic construct
  source 1..20: mol_type = other RNA
attgggcctgttaagtgatg

SEQ ID NO: 23565 - RNA, 20 nt, synthetic construct
  source 1..20: mol_type = other RNA
caggcccaataggaaacgtg

SEQ ID NO: 23566 - RNA, 20 nt, synthetic construct
  source 1..20: mol_type = other RNA
tcaaccacacgtttcctatt

SEQ ID NO: 23567 - RNA, 20 nt, synthetic construct
  source 1..20: mol_type = other RNA
atcaaccacacgtttcctat

SEQ ID NO: 23568 - RNA, 20 nt, synthetic construct
  source 1..20: mol_type = other RNA
gtgtggttgatgccccaaac

SEQ ID NO: 23569 - RNA, 20 nt, synthetic construct
  source 1..20: mol_type = other RNA
tggaatacatggcctgtttg

SEQ ID NO: 23570 - RNA, 20 nt, synthetic construct
  source 1..20: mol_type = other RNA
atggaatacatggcctgttt

SEQ ID NO: 23571 - RNA, 20 nt, synthetic construct
  source 1..20: mol_type = other RNA
tatggaatacatggcctgtt

SEQ ID NO: 23572 - RNA, 20 nt, synthetic construct
  source 1..20: mol_type = other RNA
ctagaagcatatggaataca

SEQ ID NO: 23573 - RNA, 20 nt, synthetic construct
  source 1..20: mol_type = other RNA
gaaaagacgctagaagcata

SEQ ID NO: 23574 - RNA, 20 nt, synthetic construct
  source 1..20: mol_type = other RNA
ttctaattgcatcatagatt

SEQ ID NO: 23575 - RNA, 20 nt, synthetic construct
  source 1..20: mol_type = other RNA
ttggaggatgagaaggggag

SEQ ID NO: 23576 - RNA, 20 nt, synthetic construct
  source 1..20: mol_type = other RNA
cttctcatcctccaagacat

SEQ ID NO: 23577 - RNA, 20 nt, synthetic construct
  source 1..20: mol_type = other RNA
atgtcttggaggatgagaag

SEQ ID NO: 23578 - RNA, 20 nt, synthetic construct
  source 1..20: mol_type = other RNA
tatgtcttggaggatgagaa

SEQ ID NO: 23579 - RNA, 20 nt, synthetic construct
  source 1..20: mol_type = other RNA
ctatgtcttggaggatgaga

SEQ ID NO: 23580 - RNA, 20 nt, synthetic construct
  source 1..20: mol_type = other RNA
agcaatgtcctatgtcttgg

SEQ ID NO: 23581 - RNA, 20 nt, synthetic construct
  source 1..20: mol_type = other RNA
tgcagcaatgtcctatgtct

SEQ ID NO: 23582 - RNA, 20 nt, synthetic construct
  source 1..20: mol_type = other RNA
acattgctgcaaagaactct

SEQ ID NO: 23583 - RNA, 20 nt, synthetic construct
  source 1..20: mol_type = other RNA
caaagaactcttggaaacag

SEQ ID NO: 23584 - RNA, 20 nt, synthetic construct
  source 1..20: mol_type = other RNA
tgaatgaagctgtagctcag

SEQ ID NO: 23585 - RNA, 20 nt, synthetic construct
  source 1..20: mol_type = other RNA
gaatgaagctgtagctcaga

SEQ ID NO: 23586 - RNA, 20 nt, synthetic construct
  source 1..20: mol_type = other RNA
gaagctgtagctcagaggga

SEQ ID NO: 23587 - RNA, 20 nt, synthetic construct
  source 1..20: mol_type = other RNA
aagctgtagctcagagggat

SEQ ID NO: 23588 - RNA, 20 nt, synthetic construct
  source 1..20: mol_type = other RNA
agctgtagctcagagggatg

SEQ ID NO: 23589 - RNA, 20 nt, synthetic construct
  source 1..20: mol_type = other RNA
aagaatacccatcttcaaga

SEQ ID NO: 23590 - RNA, 20 nt, synthetic construct
  source 1..20: mol_type = other RNA
aatacccatcttcaagaagg

SEQ ID NO: 23591 - RNA, 20 nt, synthetic construct
  source 1..20: mol_type = other RNA
atctccaccttcttgaagat

SEQ ID NO: 23592 - RNA, 20 nt, synthetic construct
  source 1..20: mol_type = other RNA
catctccaccttcttgaaga

SEQ ID NO: 23593 - RNA, 20 nt, synthetic construct
  source 1..20: mol_type = other RNA
catctaacccatgcttcctg

SEQ ID NO: 23594 - RNA, 20 nt, synthetic construct
  source 1..20: mol_type = other RNA
caggaagcatgggttagatg

SEQ ID NO: 23595 - RNA, 20 nt, synthetic construct
  source 1..20: mol_type = other RNA
tcaggaagcatgggttagat

SEQ ID NO: 23596 - RNA, 20 nt, synthetic construct
  source 1..20: mol_type = other RNA
ctcaggaagcatgggttaga

SEQ ID NO: 23597 - RNA, 20 nt, synthetic construct
  source 1..20: mol_type = other RNA
ccatgcttcctgaggtcatc

SEQ ID NO: 23598 - RNA, 20 nt, synthetic construct
  source 1..20: mol_type = other RNA
cagatgacctcaggaagcat

SEQ ID NO: 23599 - RNA, 20 nt, synthetic construct
  source 1..20: mol_type = other RNA
ccagatgacctcaggaagca

SEQ ID NO: 23600 - RNA, 20 nt, synthetic construct
  source 1..20: mol_type = other RNA
tgaggtcatctggactgaaa

SEQ ID NO: 23601 - RNA, 20 nt, synthetic construct
  source 1..20: mol_type = other RNA
gaggtcatctggactgaaaa

SEQ ID NO: 23602 - RNA, 20 nt, synthetic construct
  source 1..20: mol_type = other RNA
ttttcagtccagatgacctc

SEQ ID NO: 23603 - RNA, 20 nt, synthetic construct
  source 1..20: mol_type = other RNA
ctctggctgctgagggcatc

SEQ ID NO: 23604 - RNA, 20 nt, synthetic construct
  source 1..20: mol_type = other RNA
cctcagcagccagagagcag

SEQ ID NO: 23605 - RNA, 20 nt, synthetic construct
  source 1..20: mol_type = other RNA
ctctgctctctggctgctga

SEQ ID NO: 23606 - RNA, 20 nt, synthetic construct
  source 1..20: mol_type = other RNA
cctctgctctctggctgctg

SEQ ID NO: 23607 - RNA, 20 nt, synthetic construct
  source 1..20: mol_type = other RNA
gagagcagaggtctctgagc

SEQ ID NO: 23608 - RNA, 20 nt, synthetic construct
  source 1..20: mol_type = other RNA
agagcagaggtctctgagct

SEQ ID NO: 23609 - RNA, 20 nt, synthetic construct
  source 1..20: mol_type = other RNA
gctcagagacctctgctctc

SEQ ID NO: 23610 - RNA, 20 nt, synthetic construct
  source 1..20: mol_type = other RNA
tctctgagctggggtcccaa

SEQ ID NO: 23611 - RNA, 20 nt, synthetic construct
  source 1..20: mol_type = other RNA
ggggtcccaatggctgagct

SEQ ID NO: 23612 - RNA, 20 nt, synthetic construct
  source 1..20: mol_type = other RNA
atggctgagcttggagagcc

SEQ ID NO: 23613 - RNA, 20 nt, synthetic construct
  source 1..20: mol_type = other RNA
tggctgagcttggagagcct

SEQ ID NO: 23614 - RNA, 20 nt, synthetic construct
  source 1..20: mol_type = other RNA
ggctctccaagctcagccat

SEQ ID NO: 23615 - RNA, 20 nt, synthetic construct
  source 1..20: mol_type = other RNA
gagcttggagagcctgggca

SEQ ID NO: 23616 - RNA, 20 nt, synthetic construct
  source 1..20: mol_type = other RNA
gggcaaggtaatgtagacag

SEQ ID NO: 23617 - RNA, 20 nt, synthetic construct
  source 1..20: mol_type = other RNA
ggcaaggtaatgtagacaga

SEQ ID NO: 23618 - RNA, 20 nt, synthetic construct
  source 1..20: mol_type = other RNA
ctgtctacattaccttgccc

SEQ ID NO: 23619 - RNA, 20 nt, synthetic construct
  source 1..20: mol_type = other RNA
gtaatgtagacagagggttg

SEQ ID NO: 23620 - RNA, 20 nt, synthetic construct
  source 1..20: mol_type = other RNA
atgtagacagagggttgtgg

SEQ ID NO: 23621 - RNA, 20 nt, synthetic construct
  source 1..20: mol_type = other RNA
acagagggttgtggtggtct

SEQ ID NO: 23622 - RNA, 20 nt, synthetic construct
  source 1..20: mol_type = other RNA
tccgcttcatctgctgcatc

SEQ ID NO: 23623 - RNA, 20 nt, synthetic construct
  source 1..20: mol_type = other RNA
gatgcagcagatgaagcgga

SEQ ID NO: 23624 - RNA, 20 nt, synthetic construct
  source 1..20: mol_type = other RNA
gcctgatgcagcagatgaag

SEQ ID NO: 23625 - RNA, 20 nt, synthetic construct
  source 1..20: mol_type = other RNA
ctgctgcatcaggcaagtgc

SEQ ID NO: 23626 - RNA, 20 nt, synthetic construct
  source 1..20: mol_type = other RNA
caggcaagtgcaggccagcc

SEQ ID NO: 23627 - RNA, 20 nt, synthetic construct
  source 1..20: mol_type = other RNA
gcaggccagccaggacaccc

SEQ ID NO: 23628 - RNA, 20 nt, synthetic construct
  source 1..20: mol_type = other RNA
caggccagccaggacaccca

SEQ ID NO: 23629 - RNA, 20 nt, synthetic construct
  source 1..20: mol_type = other RNA
tgtgccctgggtgtcctggc

SEQ ID NO: 23630 - RNA, 20 nt, synthetic construct
  source 1..20: mol_type = other RNA
gtcttgtgccctgggtgtcc

SEQ ID NO: 23631 - RNA, 20 nt, synthetic construct
  source 1..20: mol_type = other RNA
cacccagggcacaagacaca

SEQ ID NO: 23632 - RNA, 20 nt, synthetic construct
  source 1..20: mol_type = other RNA
ggccctgtgtcttgtgccct

SEQ ID NO: 23633 - RNA, 20 nt, synthetic construct
  source 1..20: mol_type = other RNA
gggccctgtgtcttgtgccc

SEQ ID NO: 23634 - RNA, 20 nt, synthetic construct
  source 1..20: mol_type = other RNA
caaatcaaacaaagagctct

SEQ ID NO: 23635 - RNA, 20 nt, synthetic construct
  source 1..20: mol_type = other RNA
tcaaatcaaacaaagagctc

SEQ ID NO: 23636 - RNA, 20 nt, synthetic construct
  source 1..20: mol_type = other RNA
gtttgatttgaccaacctaa

SEQ ID NO: 23637 - RNA, 20 nt, synthetic construct
  source 1..20: mol_type = other RNA
agcaattagagcctttaggt

SEQ ID NO: 23638 - RNA, 20 nt, synthetic construct
  source 1..20: mol_type = other RNA
ggcaagcaattagagccttt

SEQ ID NO: 23639 - RNA, 20 nt, synthetic construct
  source 1..20: mol_type = other RNA
acagatatttcacagatgaa

SEQ ID NO: 23640 - RNA, 20 nt, synthetic construct
  source 1..20: mol_type = other RNA
gtagaaatattccttcctgc

SEQ ID NO: 23641 - RNA, 20 nt, synthetic construct
  source 1..20: mol_type = other RNA
gttctctgagtccagcagga

SEQ ID NO: 23642 - RNA, 20 nt, synthetic construct
  source 1..20: mol_type = other RNA
tgctggactcagagaacccc

SEQ ID NO: 23643 - RNA, 20 nt, synthetic construct
  source 1..20: mol_type = other RNA
tggggttctctgagtccagc

SEQ ID NO: 23644 - RNA, 20 nt, synthetic construct
  source 1..20: mol_type = other RNA
cacgttgggtagaggtcctg

SEQ ID NO: 23645 - RNA, 20 nt, synthetic construct
  source 1..20: mol_type = other RNA
gcacgttgggtagaggtcct

SEQ ID NO: 23646 - RNA, 20 nt, synthetic construct
  source 1..20: mol_type = other RNA
ggcacgttgggtagaggtcc

SEQ ID NO: 23647 - RNA, 20 nt, synthetic construct
  source 1..20: mol_type = other RNA
ggagcaggcacgttgggtag

SEQ ID NO: 23648 - RNA, 20 nt, synthetic construct
  source 1..20: mol_type = other RNA
caacgtgcctgctccaaaga

SEQ ID NO: 23649 - RNA, 20 nt, synthetic construct
  source 1..20: mol_type = other RNA
ttctttggagcaggcacgtt

SEQ ID NO: 23650 - RNA, 20 nt, synthetic construct
  source 1..20: mol_type = other RNA
cttctttggagcaggcacgt

SEQ ID NO: 23651 - RNA, 20 nt, synthetic construct
  source 1..20: mol_type = other RNA
cctgctccaaagaaggaatg

SEQ ID NO: 23652 - RNA, 20 nt, synthetic construct
  source 1..20: mol_type = other RNA
cctcattccttctttggagc

SEQ ID NO: 23653 - RNA, 20 nt, synthetic construct
  source 1..20: mol_type = other RNA
gcagaacctcattccttctt

SEQ ID NO: 23654 - RNA, 20 nt, synthetic construct
  source 1..20: mol_type = other RNA
aatgaggttctgcagagctg

SEQ ID NO: 23655 - RNA, 20 nt, synthetic construct
  source 1..20: mol_type = other RNA
ctgtggtccgagccgtgatc

SEQ ID NO: 23656 - RNA, 20 nt, synthetic construct
  source 1..20: mol_type = other RNA
ggtccgagccgtgatcagga

SEQ ID NO: 23657 - RNA, 20 nt, synthetic construct
  source 1..20: mol_type = other RNA
catccttcctgatcacggct

SEQ ID NO: 23658 - RNA, 20 nt, synthetic construct
  source 1..20: mol_type = other RNA
cgtgatcaggaaggatgcct

SEQ ID NO: 23659 - RNA, 20 nt, synthetic construct
  source 1..20: mol_type = other RNA
gtgatcaggaaggatgcctc

SEQ ID NO: 23660 - RNA, 20 nt, synthetic construct
  source 1..20: mol_type = other RNA
cgaggcatccttcctgatca

SEQ ID NO: 23661 - RNA, 20 nt, synthetic construct
  source 1..20: mol_type = other RNA
ggggaaaactatacttcccg

SEQ ID NO: 23662 - RNA, 20 nt, synthetic construct
  source 1..20: mol_type = other RNA
cactgctgggcagtttgctg

SEQ ID NO: 23663 - RNA, 20 nt, synthetic construct
  source 1..20: mol_type = other RNA
gcactgctgggcagtttgct

SEQ ID NO: 23664 - RNA, 20 nt, synthetic construct
  source 1..20: mol_type = other RNA
tgcactgctgggcagtttgc

SEQ ID NO: 23665 - RNA, 20 nt, synthetic construct
  source 1..20: mol_type = other RNA
ctgcccagcagtgcatccgc

SEQ ID NO: 23666 - RNA, 20 nt, synthetic construct
  source 1..20: mol_type = other RNA
agcagtgcatccgccggctg

SEQ ID NO: 23667 - RNA, 20 nt, synthetic construct
  source 1..20: mol_type = other RNA
cagccggcggatgcactgct

SEQ ID NO: 23668 - RNA, 20 nt, synthetic construct
  source 1..20: mol_type = other RNA
acagccggcggatgcactgc

SEQ ID NO: 23669 - RNA, 20 nt, synthetic construct
  source 1..20: mol_type = other RNA
gtgcatccgccggctgtggc

SEQ ID NO: 23670 - RNA, 20 nt, synthetic construct
  source 1..20: mol_type = other RNA
ctggagccagccacagccgg

SEQ ID NO: 23671 - RNA, 20 nt, synthetic construct
  source 1..20: mol_type = other RNA
gcactggagccagccacagc

SEQ ID NO: 23672 - RNA, 20 nt, synthetic construct
  source 1..20: mol_type = other RNA
tgcagacagagctcagaact

SEQ ID NO: 23673 - RNA, 20 nt, synthetic construct
  source 1..20: mol_type = other RNA
gttctgagctctgtctgcac

SEQ ID NO: 23674 - RNA, 20 nt, synthetic construct
  source 1..20: mol_type = other RNA
ggctcctgcaagacccatcc

SEQ ID NO: 23675 - RNA, 20 nt, synthetic construct
  source 1..20: mol_type = other RNA
tgagccaggatgggtcttgc

SEQ ID NO: 23676 - RNA, 20 nt, synthetic construct
  source 1..20: mol_type = other RNA
tggtgtagatgagccaggat

SEQ ID NO: 23677 - RNA, 20 nt, synthetic construct
  source 1..20: mol_type = other RNA
atggtgtagatgagccagga

SEQ ID NO: 23678 - RNA, 20 nt, synthetic construct
  source 1..20: mol_type = other RNA
ctcgatggtgtagatgagcc

SEQ ID NO: 23679 - RNA, 20 nt, synthetic construct
  source 1..20: mol_type = other RNA
cggctgctcttcatcctcga

SEQ ID NO: 23680 - RNA, 20 nt, synthetic construct
  source 1..20: mol_type = other RNA
aggatgaagagcagccgctc

SEQ ID NO: 23681 - RNA, 20 nt, synthetic construct
  source 1..20: mol_type = other RNA
gcagccgctctggcctagac

SEQ ID NO: 23682 - RNA, 20 nt, synthetic construct
  source 1..20: mol_type = other RNA
agatcctgtctaggccagag

SEQ ID NO: 23683 - RNA, 20 nt, synthetic construct
  source 1..20: mol_type = other RNA
cctagacaggatctgtctaa

SEQ ID NO: 23684 - RNA, 20 nt, synthetic construct
  source 1..20: mol_type = other RNA
ctagacaggatctgtctaat

SEQ ID NO: 23685 - RNA, 20 nt, synthetic construct
  source 1..20: mol_type = other RNA
ccattagacagatcctgtct

SEQ ID NO: 23686 - RNA, 20 nt, synthetic construct
  source 1..20: mol_type = other RNA
aggatctgtctaatgggagc

SEQ ID NO: 23687 - RNA, 20 nt, synthetic construct
  source 1..20: mol_type = other RNA
ctgtctaatgggagccggag

SEQ ID NO: 23688 - RNA, 20 nt, synthetic construct
  source 1..20: mol_type = other RNA
aaaagatgggacagccactc

SEQ ID NO: 23689 - RNA, 20 nt, synthetic construct
  source 1..20: mol_type = other RNA
ctgagctcatcggaaaagat

SEQ ID NO: 23690 - RNA, 20 nt, synthetic construct
  source 1..20: mol_type = other RNA
gctgagctcatcggaaaaga

SEQ ID NO: 23691 - RNA, 20 nt, synthetic construct
  source 1..20: mol_type = other RNA
gtgagtctcgctgagctcat

SEQ ID NO: 23692 - RNA, 20 nt, synthetic construct
  source 1..20: mol_type = other RNA
ctcagcgagactcaccacct

SEQ ID NO: 23693 - RNA, 20 nt, synthetic construct
  source 1..20: mol_type = other RNA
cgagactcaccaccttggac

SEQ ID NO: 23694 - RNA, 20 nt, synthetic construct
  source 1..20: mol_type = other RNA
gagactcaccaccttggact

SEQ ID NO: 23695 - RNA, 20 nt, synthetic construct
  source 1..20: mol_type = other RNA
agagctggcccagtccaagg

SEQ ID NO: 23696 - RNA, 20 nt, synthetic construct
  source 1..20: mol_type = other RNA
cagagagctggcccagtcca

SEQ ID NO: 23697 - RNA, 20 nt, synthetic construct
  source 1..20: mol_type = other RNA
ctacttcagctgcagagagc

SEQ ID NO: 23698 - RNA, 20 nt, synthetic construct
  source 1..20: mol_type = other RNA
agctgaagtagaagacatgc

SEQ ID NO: 23699 - RNA, 20 nt, synthetic construct
  source 1..20: mol_type = other RNA
agtagaagacatgctggaag

SEQ ID NO: 23700 - RNA, 20 nt, synthetic construct
  source 1..20: mol_type = other RNA
ggaagcggtccccatacagc

SEQ ID NO: 23701 - RNA, 20 nt, synthetic construct
  source 1..20: mol_type = other RNA
atacagctggcctctccccc

SEQ ID NO: 23702 - RNA, 20 nt, synthetic construct
  source 1..20: mol_type = other RNA
ggggagaggccagctgtatg

SEQ ID NO: 23703 - RNA, 20 nt, synthetic construct
  source 1..20: mol_type = other RNA
gggggagaggccagctgtat

SEQ ID NO: 23704 - RNA, 20 nt, synthetic construct
  source 1..20: mol_type = other RNA
tgggggagaggccagctgta

SEQ ID NO: 23705 - RNA, 20 nt, synthetic construct
  source 1..20: mol_type = other RNA
gtgaaggaagcctgggggag

SEQ ID NO: 23706 - RNA, 20 nt, synthetic construct
  source 1..20: mol_type = other RNA
ccaggcttccttcacctgcc

SEQ ID NO: 23707 - RNA, 20 nt, synthetic construct
  source 1..20: mol_type = other RNA
ggcaggtgaaggaagcctgg

SEQ ID NO: 23708 - RNA, 20 nt, synthetic construct
  source 1..20: mol_type = other RNA
aggcaggtgaaggaagcctg

SEQ ID NO: 23709 - RNA, 20 nt, synthetic construct
  source 1..20: mol_type = other RNA
caggcaggtgaaggaagcct

SEQ ID NO: 23710 - RNA, 20 nt, synthetic construct
  source 1..20: mol_type = other RNA
ccaggcaggtgaaggaagcc

SEQ ID NO: 23711 - RNA, 20 nt, synthetic construct
  source 1..20: mol_type = other RNA
aacactggccaggcaggtga

SEQ ID NO: 23712 - RNA, 20 nt, synthetic construct
  source 1..20: mol_type = other RNA
gaagtcaacactggccaggc

SEQ ID NO: 23713 - RNA, 20 nt, synthetic construct
  source 1..20: mol_type = other RNA
ttgggaagtcaacactggcc

SEQ ID NO: 23714 - RNA, 20 nt, synthetic construct
  source 1..20: mol_type = other RNA
tggaattgggaagtcaacac

SEQ ID NO: 23715 - RNA, 20 nt, synthetic construct
  source 1..20: mol_type = other RNA
tgcagggggctgctggaatt

SEQ ID NO: 23716 - RNA, 20 nt, synthetic construct
  source 1..20: mol_type = other RNA
ctgcagggggctgctggaat

SEQ ID NO: 23717 - RNA, 20 nt, synthetic construct
  source 1..20: mol_type = other RNA
gtcatactgcagggggctgc

SEQ ID NO: 23718 - RNA, 20 nt, synthetic construct
  source 1..20: mol_type = other RNA
ccctgcagtatgactatgcg

SEQ ID NO: 23719 - RNA, 20 nt, synthetic construct
  source 1..20: mol_type = other RNA
tcgcatagtcatactgcagg

SEQ ID NO: 23720 - RNA, 20 nt, synthetic construct
  source 1..20: mol_type = other RNA
ctcgcatagtcatactgcag

SEQ ID NO: 23721 - RNA, 20 nt, synthetic construct
  source 1..20: mol_type = other RNA
cctcgcatagtcatactgca

SEQ ID NO: 23722 - RNA, 20 nt, synthetic construct
  source 1..20: mol_type = other RNA
acctcgcatagtcatactgc

SEQ ID NO: 23723 - RNA, 20 nt, synthetic construct
  source 1..20: mol_type = other RNA
gtatgactatgcgaggttct

SEQ ID NO: 23724 - RNA, 20 nt, synthetic construct
  source 1..20: mol_type = other RNA
tatgactatgcgaggttctt

SEQ ID NO: 23725 - RNA, 20 nt, synthetic construct
  source 1..20: mol_type = other RNA
tgcgaggttcttgggtatcc

SEQ ID NO: 23726 - RNA, 20 nt, synthetic construct
  source 1..20: mol_type = other RNA
ggttcttgggtatccaggcc

SEQ ID NO: 23727 - RNA, 20 nt, synthetic construct
  source 1..20: mol_type = other RNA
gttcttgggtatccaggcct

SEQ ID NO: 23728 - RNA, 20 nt, synthetic construct
  source 1..20: mol_type = other RNA
agacttatttggcccaggcc

SEQ ID NO: 23729 - RNA, 20 nt, synthetic construct
  source 1..20: mol_type = other RNA
atcagagacttatttggccc

SEQ ID NO: 23730 - RNA, 20 nt, synthetic construct
  source 1..20: mol_type = other RNA
attgagatcagagacttatt

SEQ ID NO: 23731 - RNA, 20 nt, synthetic construct
  source 1..20: mol_type = other RNA
cgattctcctccacataatc

SEQ ID NO: 23732 - RNA, 20 nt, synthetic construct
  source 1..20: mol_type = other RNA
gattatgtggaggagaatcg

SEQ ID NO: 23733 - RNA, 20 nt, synthetic construct
  source 1..20: mol_type = other RNA
aagctggcctgattatgtgg

SEQ ID NO: 23734 - RNA, 20 nt, synthetic construct
  source 1..20: mol_type = other RNA
gagaagctggcctgattatg

SEQ ID NO: 23735 - RNA, 20 nt, synthetic construct
  source 1..20: mol_type = other RNA
caggccagcttctcttgacc

SEQ ID NO: 23736 - RNA, 20 nt, synthetic construct
  source 1..20: mol_type = other RNA
aggccagcttctcttgacca

SEQ ID NO: 23737 - RNA, 20 nt, synthetic construct
  source 1..20: mol_type = other RNA
ggccagcttctcttgaccag

SEQ ID NO: 23738 - RNA, 20 nt, synthetic construct
  source 1..20: mol_type = other RNA
atcccctggtcaagagaagc

SEQ ID NO: 23739 - RNA, 20 nt, synthetic construct
  source 1..20: mol_type = other RNA
gaccaggggatcttggcttc

SEQ ID NO: 23740 - RNA, 20 nt, synthetic construct
  source 1..20: mol_type = other RNA
accaggggatcttggcttct

SEQ ID NO: 23741 - RNA, 20 nt, synthetic construct
  source 1..20: mol_type = other RNA
ccaggggatcttggcttctg

SEQ ID NO: 23742 - RNA, 20 nt, synthetic construct
  source 1..20: mol_type = other RNA
ccccagaagccaagatcccc

SEQ ID NO: 23743 - RNA, 20 nt, synthetic construct
  source 1..20: mol_type = other RNA
gtagcagctgtgtgaatttt

SEQ ID NO: 23744 - RNA, 20 nt, synthetic construct
  source 1..20: mol_type = other RNA
gttaaaatcctcatttttcc

SEQ ID NO: 23745 - RNA, 20 nt, synthetic construct
  source 1..20: mol_type = other RNA
ttaaaatcctcatttttcca

SEQ ID NO: 23746 - RNA, 20 nt, synthetic construct
  source 1..20: mol_type = other RNA
ctcatttttccagggccatg

SEQ ID NO: 23747 - RNA, 20 nt, synthetic construct
  source 1..20: mol_type = other RNA
cacatggccctggaaaaatg

SEQ ID NO: 23748 - RNA, 20 nt, synthetic construct
  source 1..20: mol_type = other RNA
tccagggccatgtggaacag

SEQ ID NO: 23749 - RNA, 20 nt, synthetic construct
  source 1..20: mol_type = other RNA
gcctctgttccacatggccc

SEQ ID NO: 23750 - RNA, 20 nt, synthetic construct
  source 1..20: mol_type = other RNA
gagagagcctctgttccaca

SEQ ID NO: 23751 - RNA, 20 nt, synthetic construct
  source 1..20: mol_type = other RNA
cagaggctctctctcacaga

SEQ ID NO: 23752 - RNA, 20 nt, synthetic construct
  source 1..20: mol_type = other RNA
tctctcacagaaggctccca

SEQ ID NO: 23753 - RNA, 20 nt, synthetic construct
  source 1..20: mol_type = other RNA
ctctcacagaaggctcccat

SEQ ID NO: 23754 - RNA, 20 nt, synthetic construct
  source 1..20: mol_type = other RNA
tcacagaaggctcccatggg

SEQ ID NO: 23755 - RNA, 20 nt, synthetic construct
  source 1..20: mol_type = other RNA
cagaaggctcccatgggtgg

SEQ ID NO: 23756 - RNA, 20 nt, synthetic construct
  source 1..20: mol_type = other RNA
aaggctcccatgggtggtgg

SEQ ID NO: 23757 - RNA, 20 nt, synthetic construct
  source 1..20: mol_type = other RNA
aggctcccatgggtggtggt

SEQ ID NO: 23758 - RNA, 20 nt, synthetic construct
  source 1..20: mol_type = other RNA
ggctcccatgggtggtggtg

SEQ ID NO: 23759 - RNA, 20 nt, synthetic construct
  source 1..20: mol_type = other RNA
atgggtggtggtggggctgt

SEQ ID NO: 23760 - RNA, 20 nt, synthetic construct
  source 1..20: mol_type = other RNA
acagccccaccaccacccat

SEQ ID NO: 23761 - RNA, 20 nt, synthetic construct
  source 1..20: mol_type = other RNA
tacagccccaccaccaccca

SEQ ID NO: 23762 - RNA, 20 nt, synthetic construct
  source 1..20: mol_type = other RNA
gtggtggtggggctgtaggc

SEQ ID NO: 23763 - RNA, 20 nt, synthetic construct
  source 1..20: mol_type = other RNA
tgtaggctggtgtgcgcctg

SEQ ID NO: 23764 - RNA, 20 nt, synthetic construct
  source 1..20: mol_type = other RNA
gtaggctggtgtgcgcctgt

SEQ ID NO: 23765 - RNA, 20 nt, synthetic construct
  source 1..20: mol_type = other RNA
taggctggtgtgcgcctgtg

SEQ ID NO: 23766 - RNA, 20 nt, synthetic construct
  source 1..20: mol_type = other RNA
aggctggtgtgcgcctgtgg

SEQ ID NO: 23767 - RNA, 20 nt, synthetic construct
  source 1..20: mol_type = other RNA
ggtggtaggaacgcccccac

SEQ ID NO: 23768 - RNA, 20 nt, synthetic construct
  source 1..20: mol_type = other RNA
gttcctaccaccgctgccca

SEQ ID NO: 23769 - RNA, 20 nt, synthetic construct
  source 1..20: mol_type = other RNA
ttcctaccaccgctgcccat

SEQ ID NO: 23770 - RNA, 20 nt, synthetic construct
  source 1..20: mol_type = other RNA
tcctaccaccgctgcccatg

SEQ ID NO: 23771 - RNA, 20 nt, synthetic construct
  source 1..20: mol_type = other RNA
cctaccaccgctgcccatgg

SEQ ID NO: 23772 - RNA, 20 nt, synthetic construct
  source 1..20: mol_type = other RNA
cccccatgggcagcggtggt

SEQ ID NO: 23773 - RNA, 20 nt, synthetic construct
  source 1..20: mol_type = other RNA
caggcccccatgggcagcgg

SEQ ID NO: 23774 - RNA, 20 nt, synthetic construct
  source 1..20: mol_type = other RNA
aggcaggcccccatgggcag

SEQ ID NO: 23775 - RNA, 20 nt, synthetic construct
  source 1..20: mol_type = other RNA
agagaaaggcaggcccccat

SEQ ID NO: 23776 - RNA, 20 nt, synthetic construct
  source 1..20: mol_type = other RNA
cagagaaaggcaggccccca

SEQ ID NO: 23777 - RNA, 20 nt, synthetic construct
  source 1..20: mol_type = other RNA
gagagaaatcagagaaaggc

SEQ ID NO: 23778 - RNA, 20 nt, synthetic construct
  source 1..20: mol_type = other RNA
gagagagagaaatcagagaa

SEQ ID NO: 23779 - RNA, 20 nt, synthetic construct
  source 1..20: mol_type = other RNA
ctttctctgatttctaagta

SEQ ID NO: 23780 - RNA, 20 nt, synthetic construct
  source 1..20: mol_type = other RNA
tttctctgatttctaagtaa

SEQ ID NO: 23781 - RNA, 20 nt, synthetic construct
  source 1..20: mol_type = other RNA
ctctgatttctaagtaaggg

SEQ ID NO: 23782 - RNA, 20 nt, synthetic construct
  source 1..20: mol_type = other RNA
tctgatttctaagtaaggga

SEQ ID NO: 23783 - RNA, 20 nt, synthetic construct
  source 1..20: mol_type = other RNA
ctaagtaagggagggaaaga

SEQ ID NO: 23784 - RNA, 20 nt, synthetic construct
  source 1..20: mol_type = other RNA
gagggaaagaaggaacataa

SEQ ID NO: 23785 - RNA, 20 nt, synthetic construct
  source 1..20: mol_type = other RNA
attaattaaacaactgtttt

SEQ ID NO: 23786 - RNA, 20 nt, synthetic construct
  source 1..20: mol_type = other RNA
cgcagtgtgtggcttggagt

SEQ ID NO: 23787 - RNA, 20 nt, synthetic construct
  source 1..20: mol_type = other RNA
agacagcgcagtgtgtggct

SEQ ID NO: 23788 - RNA, 20 nt, synthetic construct
  source 1..20: mol_type = other RNA
tctgcagacagcgcagtgtg

SEQ ID NO: 23789 - RNA, 20 nt, synthetic construct
  source 1..20: mol_type = other RNA
actgcgctgtctgcagacac

SEQ ID NO: 23790 - RNA, 20 nt, synthetic construct
  source 1..20: mol_type = other RNA
ggcaggctaagcagaggttc

SEQ ID NO: 23791 - RNA, 20 nt, synthetic construct
  source 1..20: mol_type = other RNA
ctctgcttagcctgccaacc

SEQ ID NO: 23792 - RNA, 20 nt, synthetic construct
  source 1..20: mol_type = other RNA
caggttggcaggctaagcag

SEQ ID NO: 23793 - RNA, 20 nt, synthetic construct
  source 1..20: mol_type = other RNA
agcctgccaacctggtcccc

SEQ ID NO: 23794 - RNA, 20 nt, synthetic construct
  source 1..20: mol_type = other RNA
gcctgccaacctggtcccca

SEQ ID NO: 23795 - RNA, 20 nt, synthetic construct
  source 1..20: mol_type = other RNA
cctgccaacctggtccccag

SEQ ID NO: 23796 - RNA, 20 nt, synthetic construct
  source 1..20: mol_type = other RNA
cccctggggaccaggttggc

SEQ ID NO: 23797 - RNA, 20 nt, synthetic construct
  source 1..20: mol_type = other RNA
gagtcccctggggaccaggt

SEQ ID NO: 23798 - RNA, 20 nt, synthetic construct
  source 1..20: mol_type = other RNA
caaagagtcccctggggacc

SEQ ID NO: 23799 - RNA, 20 nt, synthetic construct
  source 1..20: mol_type = other RNA
tatggacaaagagtcccctg

SEQ ID NO: 23800 - RNA, 20 nt, synthetic construct
  source 1..20: mol_type = other RNA
gtatggacaaagagtcccct

SEQ ID NO: 23801 - RNA, 20 nt, synthetic construct
  source 1..20: mol_type = other RNA
tgtatggacaaagagtcccc

SEQ ID NO: 23802 - RNA, 20 nt, synthetic construct
  source 1..20: mol_type = other RNA
aggtgggagaggcaaatgta

SEQ ID NO: 23803 - RNA, 20 nt, synthetic construct
  source 1..20: mol_type = other RNA
tcccacctcaccaccccgcc

SEQ ID NO: 23804 - RNA, 20 nt, synthetic construct
  source 1..20: mol_type = other RNA
gcggggtggtgaggtgggag

SEQ ID NO: 23805 - RNA, 20 nt, synthetic construct
  source 1..20: mol_type = other RNA
tcctggcggggtggtgaggt

SEQ ID NO: 23806 - RNA, 20 nt, synthetic construct
  source 1..20: mol_type = other RNA
ctcctggcggggtggtgagg

SEQ ID NO: 23807 - RNA, 20 nt, synthetic construct
  source 1..20: mol_type = other RNA
gagctcctggcggggtggtg

SEQ ID NO: 23808 - RNA, 20 nt, synthetic construct
  source 1..20: mol_type = other RNA
caccccgccaggagctcagt

SEQ ID NO: 23809 - RNA, 20 nt, synthetic construct
  source 1..20: mol_type = other RNA
accccgccaggagctcagta

SEQ ID NO: 23810 - RNA, 20 nt, synthetic construct
  source 1..20: mol_type = other RNA
ctactgagctcctggcgggg

SEQ ID NO: 23811 - RNA, 20 nt, synthetic construct
  source 1..20: mol_type = other RNA
accctactgagctcctggcg

SEQ ID NO: 23812 - RNA, 20 nt, synthetic construct
  source 1..20: mol_type = other RNA
gaccctactgagctcctggc

SEQ ID NO: 23813 - RNA, 20 nt, synthetic construct
  source 1..20: mol_type = other RNA
agaccctactgagctcctgg

SEQ ID NO: 23814 - RNA, 20 nt, synthetic construct
  source 1..20: mol_type = other RNA
gtgagaccctactgagctcc

SEQ ID NO: 23815 - RNA, 20 nt, synthetic construct
  source 1..20: mol_type = other RNA
acgtcaggaatttactacac

SEQ ID NO: 23816 - RNA, 20 nt, synthetic construct
  source 1..20: mol_type = other RNA
attcctgacgtttcatccag

SEQ ID NO: 23817 - RNA, 20 nt, synthetic construct
  source 1..20: mol_type = other RNA
acgtttcatccagaggccat

SEQ ID NO: 23818 - RNA, 20 nt, synthetic construct
  source 1..20: mol_type = other RNA
tggcctctggatgaaacgtc

SEQ ID NO: 23819 - RNA, 20 nt, synthetic construct
  source 1..20: mol_type = other RNA
tccagaggccattgggtccc

SEQ ID NO: 23820 - RNA, 20 nt, synthetic construct
  source 1..20: mol_type = other RNA
tcctgggacccaatggcctc

SEQ ID NO: 23821 - RNA, 20 nt, synthetic construct
  source 1..20: mol_type = other RNA
aggaggctcctgggacccaa

SEQ ID NO: 23822 - RNA, 20 nt, synthetic construct
  source 1..20: mol_type = other RNA
cccaggagcctcctgctctc

SEQ ID NO: 23823 - RNA, 20 nt, synthetic construct
  source 1..20: mol_type = other RNA
ccaggagcctcctgctctct

SEQ ID NO: 23824 - RNA, 20 nt, synthetic construct
  source 1..20: mol_type = other RNA
ccagagagcaggaggctcct

SEQ ID NO: 23825 - RNA, 20 nt, synthetic construct
  source 1..20: mol_type = other RNA
cccagagagcaggaggctcc

SEQ ID NO: 23826 - RNA, 20 nt, synthetic construct
  source 1..20: mol_type = other RNA
cctcctgctctctgggtgct

SEQ ID NO: 23827 - RNA, 20 nt, synthetic construct
  source 1..20: mol_type = other RNA
ctgctctctgggtgctaggc

SEQ ID NO: 23828 - RNA, 20 nt, synthetic construct
  source 1..20: mol_type = other RNA
cctagcacccagagagcagg

SEQ ID NO: 23829 - RNA, 20 nt, synthetic construct
  source 1..20: mol_type = other RNA
cagcctagcacccagagagc

SEQ ID NO: 23830 - RNA, 20 nt, synthetic construct
  source 1..20: mol_type = other RNA
ctgggtgctaggctgggctg

SEQ ID NO: 23831 - RNA, 20 nt, synthetic construct
  source 1..20: mol_type = other RNA
ggtgctaggctgggctgagg

SEQ ID NO: 23832 - RNA, 20 nt, synthetic construct
  source 1..20: mol_type = other RNA
gtgctaggctgggctgaggt

SEQ ID NO: 23833 - RNA, 20 nt, synthetic construct
  source 1..20: mol_type = other RNA
tgctaggctgggctgaggtg

SEQ ID NO: 23834 - RNA, 20 nt, synthetic construct
  source 1..20: mol_type = other RNA
ccagctccccagcactgctg

SEQ ID NO: 23835 - RNA, 20 nt, synthetic construct
  source 1..20: mol_type = other RNA
acagcagtgctggggagctg

SEQ ID NO: 23836 - RNA, 20 nt, synthetic construct
  source 1..20: mol_type = other RNA
cacagcagtgctggggagct

SEQ ID NO: 23837 - RNA, 20 nt, synthetic construct
  source 1..20: mol_type = other RNA
ccacagcagtgctggggagc

SEQ ID NO: 23838 - RNA, 20 nt, synthetic construct
  source 1..20: mol_type = other RNA
ccccagcactgctgtggatg

SEQ ID NO: 23839 - RNA, 20 nt, synthetic construct
  source 1..20: mol_type = other RNA
cccagcactgctgtggatgt

SEQ ID NO: 23840 - RNA, 20 nt, synthetic construct
  source 1..20: mol_type = other RNA
ccagcactgctgtggatgtg

SEQ ID NO: 23841 - RNA, 20 nt, synthetic construct
  source 1..20: mol_type = other RNA
cagcactgctgtggatgtgg

SEQ ID NO: 23842 - RNA, 20 nt, synthetic construct
  source 1..20: mol_type = other RNA
ccacatccacagcagtgctg

SEQ ID NO: 23843 - RNA, 20 nt, synthetic construct
  source 1..20: mol_type = other RNA
cccacatccacagcagtgct

SEQ ID NO: 23844 - RNA, 20 nt, synthetic construct
  source 1..20: mol_type = other RNA
ccccacatccacagcagtgc

SEQ ID NO: 23845 - RNA, 20 nt, synthetic construct
  source 1..20: mol_type = other RNA
tgctgtggatgtgggggcgt

SEQ ID NO: 23846 - RNA, 20 nt, synthetic construct
  source 1..20: mol_type = other RNA
gctgtggatgtgggggcgtt

SEQ ID NO: 23847 - RNA, 20 nt, synthetic construct
  source 1..20: mol_type = other RNA
tgggggcgttgggtgactcc

SEQ ID NO: 23848 - RNA, 20 nt, synthetic construct
  source 1..20: mol_type = other RNA
gcgttgggtgactcctggct

SEQ ID NO: 23849 - RNA, 20 nt, synthetic construct
  source 1..20: mol_type = other RNA
actcctggcttggagactca

SEQ ID NO: 23850 - RNA, 20 nt, synthetic construct
  source 1..20: mol_type = other RNA
tggcttggagactcatggtc

SEQ ID NO: 23851 - RNA, 20 nt, synthetic construct
  source 1..20: mol_type = other RNA
ggcttggagactcatggtct

SEQ ID NO: 23852 - RNA, 20 nt, synthetic construct
  source 1..20: mol_type = other RNA
gcttggagactcatggtctg

SEQ ID NO: 23853 - RNA, 20 nt, synthetic construct
  source 1..20: mol_type = other RNA
agaccatgagtctccaagcc

SEQ ID NO: 23854 - RNA, 20 nt, synthetic construct
  source 1..20: mol_type = other RNA
gactcatggtctggggagct

SEQ ID NO: 23855 - RNA, 20 nt, synthetic construct
  source 1..20: mol_type = other RNA
ctggggagcttggaagagct

SEQ ID NO: 23856 - RNA, 20 nt, synthetic construct
  source 1..20: mol_type = other RNA
agcttggaagagcttggtag

SEQ ID NO: 23857 - RNA, 20 nt, synthetic construct
  source 1..20: mol_type = other RNA
aagagcttggtagaggagtg

SEQ ID NO: 23858 - RNA, 20 nt, synthetic construct
  source 1..20: mol_type = other RNA
aggagtgaggcagagatttc

SEQ ID NO: 23859 - RNA, 20 nt, synthetic construct
  source 1..20: mol_type = other RNA
ggagtgaggcagagatttct

SEQ ID NO: 23860 - RNA, 20 nt, synthetic construct
  source 1..20: mol_type = other RNA
gagtgaggcagagatttctg

SEQ ID NO: 23861 - RNA, 20 nt, synthetic construct
  source 1..20: mol_type = other RNA
agtgaggcagagatttctgg

SEQ ID NO: 23862 - RNA, 20 nt, synthetic construct
  source 1..20: mol_type = other RNA
gtgaggcagagatttctggg

SEQ ID NO: 23863 - RNA, 20 nt, synthetic construct
  source 1..20: mol_type = other RNA
gaaaataaatgttcagtaaa

SEQ ID NO: 23864 - RNA, 20 nt, synthetic construct
  source 1..20: mol_type = other RNA
ctgaacatttattttctttt

SEQ ID NO: 23865 - RNA, 20 nt, synthetic construct
  source 1..20: mol_type = other RNA
ctcacaacagtcctgagaga

SEQ ID NO: 23866 - RNA, 20 nt, synthetic construct
  source 1..20: mol_type = other RNA
tcacaacagtcctgagagat

SEQ ID NO: 23867 - RNA, 20 nt, synthetic construct
  source 1..20: mol_type = other RNA
attattaagacccatctctc

SEQ ID NO: 23868 - RNA, 20 nt, synthetic construct
  source 1..20: mol_type = other RNA
ggacagcagaggaaggatag

SEQ ID NO: 23869 - RNA, 20 nt, synthetic construct
  source 1..20: mol_type = other RNA
gggacagcagaggaaggata

SEQ ID NO: 23870 - RNA, 20 nt, synthetic construct
  source 1..20: mol_type = other RNA
ggggacagcagaggaaggat

SEQ ID NO: 23871 - RNA, 20 nt, synthetic construct
  source 1..20: mol_type = other RNA
cctctgctgtcccccatgtc

SEQ ID NO: 23872 - RNA, 20 nt, synthetic construct
  source 1..20: mol_type = other RNA
acatgggggacagcagagga

SEQ ID NO: 23873 - RNA, 20 nt, synthetic construct
  source 1..20: mol_type = other RNA
cctgacatgggggacagcag

SEQ ID NO: 23874 - RNA, 20 nt, synthetic construct
  source 1..20: mol_type = other RNA
tgcatggggacctgacatgg

SEQ ID NO: 23875 - RNA, 20 nt, synthetic construct
  source 1..20: mol_type = other RNA
gtgcatggggacctgacatg

SEQ ID NO: 23876 - RNA, 20 nt, synthetic construct
  source 1..20: mol_type = other RNA
tgtgcatggggacctgacat

SEQ ID NO: 23877 - RNA, 20 nt, synthetic construct
  source 1..20: mol_type = other RNA
ctgtgcatggggacctgaca

SEQ ID NO: 23878 - RNA, 20 nt, synthetic construct
  source 1..20: mol_type = other RNA
catgcacagacatgatcctc

SEQ ID NO: 23879 - RNA, 20 nt, synthetic construct
  source 1..20: mol_type = other RNA
atgcacagacatgatcctct

SEQ ID NO: 23880 - RNA, 20 nt, synthetic construct
  source 1..20: mol_type = other RNA
gaggatcatgtctgtgcatg

SEQ ID NO: 23881 - RNA, 20 nt, synthetic construct
  source 1..20: mol_type = other RNA
agaggatcatgtctgtgcat

SEQ ID NO: 23882 - RNA, 20 nt, synthetic construct
  source 1..20: mol_type = other RNA
cacagacatgatcctctggg

SEQ ID NO: 23883 - RNA, 20 nt, synthetic construct
  source 1..20: mol_type = other RNA
acagacatgatcctctgggt

SEQ ID NO: 23884 - RNA, 20 nt, synthetic construct
  source 1..20: mol_type = other RNA
cagacatgatcctctgggtg

SEQ ID NO: 23885 - RNA, 20 nt, synthetic construct
  source 1..20: mol_type = other RNA
agctggtgggccccacccag

SEQ ID NO: 23886 - RNA, 20 nt, synthetic construct
  source 1..20: mol_type = other RNA
ggagctgtgaatcagctggt

SEQ ID NO: 23887 - RNA, 20 nt, synthetic construct
  source 1..20: mol_type = other RNA
tggagctgtgaatcagctgg

SEQ ID NO: 23888 - RNA, 20 nt, synthetic construct
  source 1..20: mol_type = other RNA
gctgattcacagctccaccc

SEQ ID NO: 23889 - RNA, 20 nt, synthetic construct
  source 1..20: mol_type = other RNA
ctgattcacagctccaccca

SEQ ID NO: 23890 - RNA, 20 nt, synthetic construct
  source 1..20: mol_type = other RNA
gggtggagctgtgaatcagc

SEQ ID NO: 23891 - RNA, 20 nt, synthetic construct
  source 1..20: mol_type = other RNA
ggcaggctgacagccctggg

SEQ ID NO: 23892 - RNA, 20 nt, synthetic construct
  source 1..20: mol_type = other RNA
tgaggcaggctgacagccct

SEQ ID NO: 23893 - RNA, 20 nt, synthetic construct
  source 1..20: mol_type = other RNA
ctgaggcaggctgacagccc

SEQ ID NO: 23894 - RNA, 20 nt, synthetic construct
  source 1..20: mol_type = other RNA
gaggtgaggcttgctgaggc

SEQ ID NO: 23895 - RNA, 20 nt, synthetic construct
  source 1..20: mol_type = other RNA
agcaagcctcacctctccag

SEQ ID NO: 23896 - RNA, 20 nt, synthetic construct
  source 1..20: mol_type = other RNA
tggagaggtgaggcttgctg

SEQ ID NO: 23897 - RNA, 20 nt, synthetic construct
  source 1..20: mol_type = other RNA
tggacgccgctggagaggtg

SEQ ID NO: 23898 - RNA, 20 nt, synthetic construct
  source 1..20: mol_type = other RNA
acatctggacgccgctggag

SEQ ID NO: 23899 - RNA, 20 nt, synthetic construct
  source 1..20: mol_type = other RNA
cagcggcgtccagatgtgtc

SEQ ID NO: 23900 - RNA, 20 nt, synthetic construct
  source 1..20: mol_type = other RNA
ctgacacatctggacgccgc

SEQ ID NO: 23901 - RNA, 20 nt, synthetic construct
  source 1..20: mol_type = other RNA
agacagctgcctgacacatc

SEQ ID NO: 23902 - RNA, 20 nt, synthetic construct
  source 1..20: mol_type = other RNA
aaacccttctctctgagccc

SEQ ID NO: 23903 - RNA, 20 nt, synthetic construct
  source 1..20: mol_type = other RNA
aacccttctctctgagccct

SEQ ID NO: 23904 - RNA, 20 nt, synthetic construct
  source 1..20: mol_type = other RNA
cacccagggctcagagagaa

SEQ ID NO: 23905 - RNA, 20 nt, synthetic construct
  source 1..20: mol_type = other RNA
gcacccagggctcagagaga

SEQ ID NO: 23906 - RNA, 20 nt, synthetic construct
  source 1..20: mol_type = other RNA
gagccctgggtgcaccccgc

SEQ ID NO: 23907 - RNA, 20 nt, synthetic construct
  source 1..20: mol_type = other RNA
ttgccggcggggtgcaccca

SEQ ID NO: 23908 - RNA, 20 nt, synthetic construct
  source 1..20: mol_type = other RNA
attgccggcggggtgcaccc

SEQ ID NO: 23909 - RNA, 20 nt, synthetic construct
  source 1..20: mol_type = other RNA
tgcaccccgccggcaattca

SEQ ID NO: 23910 - RNA, 20 nt, synthetic construct
  source 1..20: mol_type = other RNA
cgccggcaattcatggatcc

SEQ ID NO: 23911 - RNA, 20 nt, synthetic construct
  source 1..20: mol_type = other RNA
gccggcaattcatggatcca

SEQ ID NO: 23912 - RNA, 20 nt, synthetic construct
  source 1..20: mol_type = other RNA
ggatccatgaattgccggcg

SEQ ID NO: 23913 - RNA, 20 nt, synthetic construct
  source 1..20: mol_type = other RNA
tggatccatgaattgccggc

SEQ ID NO: 23914 - RNA, 20 nt, synthetic construct
  source 1..20: mol_type = other RNA
ctggatccatgaattgccgg

SEQ ID NO: 23915 - RNA, 20 nt, synthetic construct
  source 1..20: mol_type = other RNA
gccctggatccatgaattgc

SEQ ID NO: 23916 - RNA, 20 nt, synthetic construct
  source 1..20: mol_type = other RNA
gatccagggcattagcactg

SEQ ID NO: 23917 - RNA, 20 nt, synthetic construct
  source 1..20: mol_type = other RNA
ccagggcattagcactgcgg

SEQ ID NO: 23918 - RNA, 20 nt, synthetic construct
  source 1..20: mol_type = other RNA
gggcattagcactgcggtgg

SEQ ID NO: 23919 - RNA, 20 nt, synthetic construct
  source 1..20: mol_type = other RNA
ccaccgcagtgctaatgccc

SEQ ID NO: 23920 - RNA, 20 nt, synthetic construct
  source 1..20: mol_type = other RNA
cattagcactgcggtggagg

SEQ ID NO: 23921 - RNA, 20 nt, synthetic construct
  source 1..20: mol_type = other RNA
attagcactgcggtggaggt

SEQ ID NO: 23922 - RNA, 20 nt, synthetic construct
  source 1..20: mol_type = other RNA
gcactgcggtggaggtgggt

SEQ ID NO: 23923 - RNA, 20 nt, synthetic construct
  source 1..20: mol_type = other RNA
tgcggtggaggtgggttggc

SEQ ID NO: 23924 - RNA, 20 nt, synthetic construct
  source 1..20: mol_type = other RNA
gcggtggaggtgggttggct

SEQ ID NO: 23925 - RNA, 20 nt, synthetic construct
  source 1..20: mol_type = other RNA
tgggttggctgggagacccc

SEQ ID NO: 23926 - RNA, 20 nt, synthetic construct
  source 1..20: mol_type = other RNA
gttggctgggagaccccagg

SEQ ID NO: 23927 - RNA, 20 nt, synthetic construct
  source 1..20: mol_type = other RNA
ttggctgggagaccccaggt

SEQ ID NO: 23928 - RNA, 20 nt, synthetic construct
  source 1..20: mol_type = other RNA
tggctgggagaccccaggtg

SEQ ID NO: 23929 - RNA, 20 nt, synthetic construct
  source 1..20: mol_type = other RNA
gaccccaggtggggttcact

SEQ ID NO: 23930 - RNA, 20 nt, synthetic construct
  source 1..20: mol_type = other RNA
accccaggtggggttcactt

SEQ ID NO: 23931 - RNA, 20 nt, synthetic construct
  source 1..20: mol_type = other RNA
gcccaagtgaaccccacctg

SEQ ID NO: 23932 - RNA, 20 nt, synthetic construct
  source 1..20: mol_type = other RNA
agcccaagtgaaccccacct

SEQ ID NO: 23933 - RNA, 20 nt, synthetic construct
  source 1..20: mol_type = other RNA
cagcccaagtgaaccccacc

SEQ ID NO: 23934 - RNA, 20 nt, synthetic construct
  source 1..20: mol_type = other RNA
ggggttcacttgggctgtag

SEQ ID NO: 23935 - RNA, 20 nt, synthetic construct
  source 1..20: mol_type = other RNA
acttgggctgtaggggaatg

SEQ ID NO: 23936 - RNA, 20 nt, synthetic construct
  source 1..20: mol_type = other RNA
cttgggctgtaggggaatga

SEQ ID NO: 23937 - RNA, 20 nt, synthetic construct
  source 1..20: mol_type = other RNA
tgtaggggaatgagggagag

SEQ ID NO: 23938 - RNA, 20 nt, synthetic construct
  source 1..20: mol_type = other RNA
aatgagggagagtggcctac

SEQ ID NO: 23939 - RNA, 20 nt, synthetic construct
  source 1..20: mol_type = other RNA
cctacaggaaagagacaaag

SEQ ID NO: 23940 - RNA, 20 nt, synthetic construct
  source 1..20: mol_type = other RNA
caggaaagagacaaagaggt

SEQ ID NO: 23941 - RNA, 20 nt, synthetic construct
  source 1..20: mol_type = other RNA
cctctttgtctctttcctgt

SEQ ID NO: 23942 - RNA, 20 nt, synthetic construct
  source 1..20: mol_type = other RNA
agaggttggagacacatcag

SEQ ID NO: 23943 - RNA, 20 nt, synthetic construct
  source 1..20: mol_type = other RNA
gaggttggagacacatcaga

SEQ ID NO: 23944 - RNA, 20 nt, synthetic construct
  source 1..20: mol_type = other RNA
aggttggagacacatcagag

SEQ ID NO: 23945 - RNA, 20 nt, synthetic construct
  source 1..20: mol_type = other RNA
tggagacacatcagaggggc

SEQ ID NO: 23946 - RNA, 20 nt, synthetic construct
  source 1..20: mol_type = other RNA
ggagacacatcagaggggca

SEQ ID NO: 23947 - RNA, 20 nt, synthetic construct
  source 1..20: mol_type = other RNA
gagacacatcagaggggcag

SEQ ID NO: 23948 - RNA, 20 nt, synthetic construct
  source 1..20: mol_type = other RNA
acatcagaggggcaggggca

SEQ ID NO: 23949 - RNA, 20 nt, synthetic construct
  source 1..20: mol_type = other RNA
aggggcaggggcaaggtgcc

SEQ ID NO: 23950 - RNA, 20 nt, synthetic construct
  source 1..20: mol_type = other RNA
ggggcaggggcaaggtgcca

SEQ ID NO: 23951 - RNA, 20 nt, synthetic construct
  source 1..20: mol_type = other RNA
aaggtgccagggaactgagc

SEQ ID NO: 23952 - RNA, 20 nt, synthetic construct
  source 1..20: mol_type = other RNA
aggagaccagctcagttccc

SEQ ID NO: 23953 - RNA, 20 nt, synthetic construct
  source 1..20: mol_type = other RNA
tctcctctctcaaccaagag

SEQ ID NO: 23954 - RNA, 20 nt, synthetic construct
  source 1..20: mol_type = other RNA
tctctcaaccaagagaggtc

SEQ ID NO: 23955 - RNA, 20 nt, synthetic construct
  source 1..20: mol_type = other RNA
tgacctctcttggttgagag

SEQ ID NO: 23956 - RNA, 20 nt, synthetic construct
  source 1..20: mol_type = other RNA
tggtgtatcctgacctctct

SEQ ID NO: 23957 - RNA, 20 nt, synthetic construct
  source 1..20: mol_type = other RNA
ccatgtcactgctcagagga

SEQ ID NO: 23958 - RNA, 20 nt, synthetic construct
  source 1..20: mol_type = other RNA
tcactgctcagaggaaggcc

SEQ ID NO: 23959 - RNA, 20 nt, synthetic construct
  source 1..20: mol_type = other RNA
tgctcagaggaaggcctggc

SEQ ID NO: 23960 - RNA, 20 nt, synthetic construct
  source 1..20: mol_type = other RNA
gctcagaggaaggcctggca

SEQ ID NO: 23961 - RNA, 20 nt, synthetic construct
  source 1..20: mol_type = other RNA
cagaggaaggcctggcaggg

SEQ ID NO: 23962 - RNA, 20 nt, synthetic construct
  source 1..20: mol_type = other RNA
agaggaaggcctggcaggga

SEQ ID NO: 23963 - RNA, 20 nt, synthetic construct
  source 1..20: mol_type = other RNA
gcctggcagggagggctcag

SEQ ID NO: 23964 - RNA, 20 nt, synthetic construct
  source 1..20: mol_type = other RNA
tggcagggagggctcagtgg

SEQ ID NO: 23965 - RNA, 20 nt, synthetic construct
  source 1..20: mol_type = other RNA
ggcagggagggctcagtggt

SEQ ID NO: 23966 - RNA, 20 nt, synthetic construct
  source 1..20: mol_type = other RNA
gcagggagggctcagtggtg

SEQ ID NO: 23967 - RNA, 20 nt, synthetic construct
  source 1..20: mol_type = other RNA
accactgagccctccctgcc

SEQ ID NO: 23968 - RNA, 20 nt, synthetic construct
  source 1..20: mol_type = other RNA
ctcagtggtggggtcccaag

SEQ ID NO: 23969 - RNA, 20 nt, synthetic construct
  source 1..20: mol_type = other RNA
tcagtggtggggtcccaaga

SEQ ID NO: 23970 - RNA, 20 nt, synthetic construct
  source 1..20: mol_type = other RNA
tggtggggtcccaagagggc

SEQ ID NO: 23971 - RNA, 20 nt, synthetic construct
  source 1..20: mol_type = other RNA
ggtggggtcccaagagggca

SEQ ID NO: 23972 - RNA, 20 nt, synthetic construct
  source 1..20: mol_type = other RNA
gggtcccaagagggcagggc

SEQ ID NO: 23973 - RNA, 20 nt, synthetic construct
  source 1..20: mol_type = other RNA
aagagggcagggcaggcatg

SEQ ID NO: 23974 - RNA, 20 nt, synthetic construct
  source 1..20: mol_type = other RNA
agagggcagggcaggcatga

SEQ ID NO: 23975 - RNA, 20 nt, synthetic construct
  source 1..20: mol_type = other RNA
catgcctgccctgccctctt

SEQ ID NO: 23976 - RNA, 20 nt, synthetic construct
  source 1..20: mol_type = other RNA
tcatgcctgccctgccctct

SEQ ID NO: 23977 - RNA, 20 nt, synthetic construct
  source 1..20: mol_type = other RNA
gcagggcaggcatgagggcc

SEQ ID NO: 23978 - RNA, 20 nt, synthetic construct
  source 1..20: mol_type = other RNA
cagggcaggcatgagggcca

SEQ ID NO: 23979 - RNA, 20 nt, synthetic construct
  source 1..20: mol_type = other RNA
agggcaggcatgagggccag

SEQ ID NO: 23980 - RNA, 20 nt, synthetic construct
  source 1..20: mol_type = other RNA
gagggccaggggatgtcccg

SEQ ID NO: 23981 - RNA, 20 nt, synthetic construct
  source 1..20: mol_type = other RNA
agggccaggggatgtcccgc

SEQ ID NO: 23982 - RNA, 20 nt, synthetic construct
  source 1..20: mol_type = other RNA
aggggatgtcccgcgggcag

SEQ ID NO: 23983 - RNA, 20 nt, synthetic construct
  source 1..20: mol_type = other RNA
ggggatgtcccgcgggcagt

SEQ ID NO: 23984 - RNA, 20 nt, synthetic construct
  source 1..20: mol_type = other RNA
gggatgtcccgcgggcagtg

SEQ ID NO: 23985 - RNA, 20 nt, synthetic construct
  source 1..20: mol_type = other RNA
actgcccgcgggacatcccc

SEQ ID NO: 23986 - RNA, 20 nt, synthetic construct
  source 1..20: mol_type = other RNA
cagaggaccccactgcccgc

SEQ ID NO: 23987 - RNA, 20 nt, synthetic construct
  source 1..20: mol_type = other RNA
acagaggaccccactgcccg

SEQ ID NO: 23988 - RNA, 20 nt, synthetic construct
  source 1..20: mol_type = other RNA
aggggcaggtgagtggacag

SEQ ID NO: 23989 - RNA, 20 nt, synthetic construct
  source 1..20: mol_type = other RNA
tccactcacctgccccttcc

SEQ ID NO: 23990 - RNA, 20 nt, synthetic construct
  source 1..20: mol_type = other RNA
ccactcacctgccccttcct

SEQ ID NO: 23991 - RNA, 20 nt, synthetic construct
  source 1..20: mol_type = other RNA
cccaggaaggggcaggtgag

SEQ ID NO: 23992 - RNA, 20 nt, synthetic construct
  source 1..20: mol_type = other RNA
acctgccccttcctgggctt

SEQ ID NO: 23993 - RNA, 20 nt, synthetic construct
  source 1..20: mol_type = other RNA
gcccaagcccaggaaggggc

SEQ ID NO: 23994 - RNA, 20 nt, synthetic construct
  source 1..20: mol_type = other RNA
gtgcgcccaagcccaggaag

SEQ ID NO: 23995 - RNA, 20 nt, synthetic construct
  source 1..20: mol_type = other RNA
tgtgcgcccaagcccaggaa

SEQ ID NO: 23996 - RNA, 20 nt, synthetic construct
  source 1..20: mol_type = other RNA
ctgtgcgcccaagcccagga

SEQ ID NO: 23997 - RNA, 20 nt, synthetic construct
  source 1..20: mol_type = other RNA
gtcactgtgcgcccaagccc

SEQ ID NO: 23998 - RNA, 20 nt, synthetic construct
  source 1..20: mol_type = other RNA
cctcagccccatctgctccc

SEQ ID NO: 23999 - RNA, 20 nt, synthetic construct
  source 1..20: mol_type = other RNA
cctgggagcagatggggctg

SEQ ID NO: 24000 - RNA, 20 nt, synthetic construct
  source 1..20: mol_type = other RNA
ccatctgctcccaggtatgg

SEQ ID NO: 24001 - RNA, 20 nt, synthetic construct
  source 1..20: mol_type = other RNA
catctgctcccaggtatgga

SEQ ID NO: 24002 - RNA, 20 nt, synthetic construct
  source 1..20: mol_type = other RNA
tccatacctgggagcagatg

SEQ ID NO: 24003 - RNA, 20 nt, synthetic construct
  source 1..20: mol_type = other RNA
ctccatacctgggagcagat

SEQ ID NO: 24004 - RNA, 20 nt, synthetic construct
  source 1..20: mol_type = other RNA
cctccatacctgggagcaga

SEQ ID NO: 24005 - RNA, 20 nt, synthetic construct
  source 1..20: mol_type = other RNA
gctcccaggtatggagggct

SEQ ID NO: 24006 - RNA, 20 nt, synthetic construct
  source 1..20: mol_type = other RNA
ggtatggagggctaggtccc

SEQ ID NO: 24007 - RNA, 20 nt, synthetic construct
  source 1..20: mol_type = other RNA
ggacctagccctccatacct

SEQ ID NO: 24008 - RNA, 20 nt, synthetic construct
  source 1..20: mol_type = other RNA
gggacctagccctccatacc

SEQ ID NO: 24009 - RNA, 20 nt, synthetic construct
  source 1..20: mol_type = other RNA
gtatggggagcagcgggcct

SEQ ID NO: 24010 - RNA, 20 nt, synthetic construct
  source 1..20: mol_type = other RNA
agtatggggagcagcgggcc

SEQ ID NO: 24011 - RNA, 20 nt, synthetic construct
  source 1..20: mol_type = other RNA
ggctcagtatggggagcagc

SEQ ID NO: 24012 - RNA, 20 nt, synthetic construct
  source 1..20: mol_type = other RNA
tggctcagtatggggagcag

SEQ ID NO: 24013 - RNA, 20 nt, synthetic construct
  source 1..20: mol_type = other RNA
atactgagccaccaggtacg

SEQ ID NO: 24014 - RNA, 20 nt, synthetic construct
  source 1..20: mol_type = other RNA
gtacctggtggctcagtatg

SEQ ID NO: 24015 - RNA, 20 nt, synthetic construct
  source 1..20: mol_type = other RNA
cgtacctggtggctcagtat

SEQ ID NO: 24016 - RNA, 20 nt, synthetic construct
  source 1..20: mol_type = other RNA
tcgtacctggtggctcagta

SEQ ID NO: 24017 - RNA, 20 nt, synthetic construct
  source 1..20: mol_type = other RNA
ggaggtggcctcgtacctgg

SEQ ID NO: 24018 - RNA, 20 nt, synthetic construct
  source 1..20: mol_type = other RNA
catggaggtggcctcgtacc

SEQ ID NO: 24019 - RNA, 20 nt, synthetic construct
  source 1..20: mol_type = other RNA
gaagacgagtggcatggagg

SEQ ID NO: 24020 - RNA, 20 nt, synthetic construct
  source 1..20: mol_type = other RNA
agagaagacgagtggcatgg

SEQ ID NO: 24021 - RNA, 20 nt, synthetic construct
  source 1..20: mol_type = other RNA
gccagagaagacgagtggca

SEQ ID NO: 24022 - RNA, 20 nt, synthetic construct
  source 1..20: mol_type = other RNA
actcgtcttctctggctgag

SEQ ID NO: 24023 - RNA, 20 nt, synthetic construct
  source 1..20: mol_type = other RNA
ctcgtcttctctggctgagc

SEQ ID NO: 24024 - RNA, 20 nt, synthetic construct
  source 1..20: mol_type = other RNA
gctcagccagagaagacgag

SEQ ID NO: 24025 - RNA, 20 nt, synthetic construct
  source 1..20: mol_type = other RNA
tgtctcacccgaagagctcc

SEQ ID NO: 24026 - RNA, 20 nt, synthetic construct
  source 1..20: mol_type = other RNA
gcgcactccaggagctcttc

SEQ ID NO: 24027 - RNA, 20 nt, synthetic construct
  source 1..20: mol_type = other RNA
agcgcactccaggagctctt

SEQ ID NO: 24028 - RNA, 20 nt, synthetic construct
  source 1..20: mol_type = other RNA
gctcctggagtgcgctttat

SEQ ID NO: 24029 - RNA, 20 nt, synthetic construct
  source 1..20: mol_type = other RNA
tcgccaataaagcgcactcc

SEQ ID NO: 24030 - RNA, 20 nt, synthetic construct
  source 1..20: mol_type = other RNA
ctttattggcgagcagaagc

SEQ ID NO: 24031 - RNA, 20 nt, synthetic construct
  source 1..20: mol_type = other RNA
ccttcagctcctccttcttc

SEQ ID NO: 24032 - RNA, 20 nt, synthetic construct
  source 1..20: mol_type = other RNA
cctgaagaaggaggagctga

SEQ ID NO: 24033 - RNA, 20 nt, synthetic construct
  source 1..20: mol_type = other RNA
cttggagttcctgaagaagg

SEQ ID NO: 24034 - RNA, 20 nt, synthetic construct
  source 1..20: mol_type = other RNA
cttcaggaactccaagtaac

SEQ ID NO: 24035 - RNA, 20 nt, synthetic construct
  source 1..20: mol_type = other RNA
ttacttggagttcctgaaga

SEQ ID NO: 24036 - RNA, 20 nt, synthetic construct
  source 1..20: mol_type = other RNA
ggaactccaagtaacaggcc

SEQ ID NO: 24037 - RNA, 20 nt, synthetic construct
  source 1..20: mol_type = other RNA
actccaagtaacaggccagg

SEQ ID NO: 24038 - RNA, 20 nt, synthetic construct
  source 1..20: mol_type = other RNA
gtaacaggccaggcggcccc

SEQ ID NO: 24039 - RNA, 20 nt, synthetic construct
  source 1..20: mol_type = other RNA
gggccgcctggcctgttact

SEQ ID NO: 24040 - RNA, 20 nt, synthetic construct
  source 1..20: mol_type = other RNA
tggcggagcctggggccgcc

SEQ ID NO: 24041 - RNA, 20 nt, synthetic construct
  source 1..20: mol_type = other RNA
gagatggctggcggagcctg

SEQ ID NO: 24042 - RNA, 20 nt, synthetic construct
  source 1..20: mol_type = other RNA
agagatggctggcggagcct

SEQ ID NO: 24043 - RNA, 20 nt, synthetic construct
  source 1..20: mol_type = other RNA
cagagatggctggcggagcc

SEQ ID NO: 24044 - RNA, 20 nt, synthetic construct
  source 1..20: mol_type = other RNA
tccgccagccatctctgtcc

SEQ ID NO: 24045 - RNA, 20 nt, synthetic construct
  source 1..20: mol_type = other RNA
tccgggacagagatggctgg

SEQ ID NO: 24046 - RNA, 20 nt, synthetic construct
  source 1..20: mol_type = other RNA
aactccgggacagagatggc

SEQ ID NO: 24047 - RNA, 20 nt, synthetic construct
  source 1..20: mol_type = other RNA
atctctgtcccggagttaag

SEQ ID NO: 24048 - RNA, 20 nt, synthetic construct
  source 1..20: mol_type = other RNA
tctctgtcccggagttaaga

SEQ ID NO: 24049 - RNA, 20 nt, synthetic construct
  source 1..20: mol_type = other RNA
tcttaactccgggacagaga

SEQ ID NO: 24050 - RNA, 20 nt, synthetic construct
  source 1..20: mol_type = other RNA
cccggagttaagagggtgtc

SEQ ID NO: 24051 - RNA, 20 nt, synthetic construct
  source 1..20: mol_type = other RNA
ccggagttaagagggtgtct

SEQ ID NO: 24052 - RNA, 20 nt, synthetic construct
  source 1..20: mol_type = other RNA
cggagttaagagggtgtctg

SEQ ID NO: 24053 - RNA, 20 nt, synthetic construct
  source 1..20: mol_type = other RNA
ggagttaagagggtgtctgg

SEQ ID NO: 24054 - RNA, 20 nt, synthetic construct
  source 1..20: mol_type = other RNA
ccagacaccctcttaactcc

SEQ ID NO: 24055 - RNA, 20 nt, synthetic construct
  source 1..20: mol_type = other RNA
cccagacaccctcttaactc

SEQ ID NO: 24056 - RNA, 20 nt, synthetic construct
  source 1..20: mol_type = other RNA
ggtgtctgggggatgttccc

SEQ ID NO: 24057 - RNA, 20 nt, synthetic construct
  source 1..20: mol_type = other RNA
gtctgggggatgttcccagg

SEQ ID NO: 24058 - RNA, 20 nt, synthetic construct
  source 1..20: mol_type = other RNA
ggggatgttcccaggtggtg

SEQ ID NO: 24059 - RNA, 20 nt, synthetic construct
  source 1..20: mol_type = other RNA
gggatgttcccaggtggtga

SEQ ID NO: 24060 - RNA, 20 nt, synthetic construct
  source 1..20: mol_type = other RNA
tcccaggtggtgagggtatc

SEQ ID NO: 24061 - RNA, 20 nt, synthetic construct
  source 1..20: mol_type = other RNA
aggtggtgagggtatcaggc

SEQ ID NO: 24062 - RNA, 20 nt, synthetic construct
  source 1..20: mol_type = other RNA
gcctgataccctcaccacct

SEQ ID NO: 24063 - RNA, 20 nt, synthetic construct
  source 1..20: mol_type = other RNA
tgcctgataccctcaccacc

SEQ ID NO: 24064 - RNA, 20 nt, synthetic construct
  source 1..20: mol_type = other RNA
aacagtgctgtcctttgcct

SEQ ID NO: 24065 - RNA, 20 nt, synthetic construct
  source 1..20: mol_type = other RNA
gacggtaagagccaaggcaa

SEQ ID NO: 24066 - RNA, 20 nt, synthetic construct
  source 1..20: mol_type = other RNA
ataagagacggtaagagcca

SEQ ID NO: 24067 - RNA, 20 nt, synthetic construct
  source 1..20: mol_type = other RNA
accgtctcttattcagcatt

SEQ ID NO: 24068 - RNA, 20 nt, synthetic construct
  source 1..20: mol_type = other RNA
tccgaatgctgaataagaga

SEQ ID NO: 24069 - RNA, 20 nt, synthetic construct
  source 1..20: mol_type = other RNA
aacccagttttataaatccc

SEQ ID NO: 24070 - RNA, 20 nt, synthetic construct
  source 1..20: mol_type = other RNA
acccagttttataaatccca

SEQ ID NO: 24071 - RNA, 20 nt, synthetic construct
  source 1..20: mol_type = other RNA
gccctgggatttataaaact

SEQ ID NO: 24072 - RNA, 20 nt, synthetic construct
  source 1..20: mol_type = other RNA
tgccctgggatttataaaac

SEQ ID NO: 24073 - RNA, 20 nt, synthetic construct
  source 1..20: mol_type = other RNA
cgtctatctgtaggtgccct

SEQ ID NO: 24074 - RNA, 20 nt, synthetic construct
  source 1..20: mol_type = other RNA
gcgtctatctgtaggtgccc

SEQ ID NO: 24075 - RNA, 20 nt, synthetic construct
  source 1..20: mol_type = other RNA
ctacagatagacgccgatag

SEQ ID NO: 24076 - RNA, 20 nt, synthetic construct
  source 1..20: mol_type = other RNA
tacagatagacgccgataga

SEQ ID NO: 24077 - RNA, 20 nt, synthetic construct
  source 1..20: mol_type = other RNA
acagatagacgccgatagag

SEQ ID NO: 24078 - RNA, 20 nt, synthetic construct
  source 1..20: mol_type = other RNA
cagatagacgccgatagagg

SEQ ID NO: 24079 - RNA, 20 nt, synthetic construct
  source 1..20: mol_type = other RNA
ctctatcggcgtctatctgt

SEQ ID NO: 24080 - RNA, 20 nt, synthetic construct
  source 1..20: mol_type = other RNA
agacgccgatagagggggag

SEQ ID NO: 24081 - RNA, 20 nt, synthetic construct
  source 1..20: mol_type = other RNA
gccgatagagggggagtggt

SEQ ID NO: 24082 - RNA, 20 nt, synthetic construct
  source 1..20: mol_type = other RNA
tcctaccactccccctctat

SEQ ID NO: 24083 - RNA, 20 nt, synthetic construct
  source 1..20: mol_type = other RNA
ggggagtggtaggaaaagcc

SEQ ID NO: 24084 - RNA, 20 nt, synthetic construct
  source 1..20: mol_type = other RNA
gggagtggtaggaaaagcca

SEQ ID NO: 24085 - RNA, 20 nt, synthetic construct
  source 1..20: mol_type = other RNA
ggagtggtaggaaaagccag

SEQ ID NO: 24086 - RNA, 20 nt, synthetic construct
  source 1..20: mol_type = other RNA
gtggtaggaaaagccagggg

SEQ ID NO: 24087 - RNA, 20 nt, synthetic construct
  source 1..20: mol_type = other RNA
tggtaggaaaagccagggga

SEQ ID NO: 24088 - RNA, 20 nt, synthetic construct
  source 1..20: mol_type = other RNA
taggaaaagccaggggaggg

SEQ ID NO: 24089 - RNA, 20 nt, synthetic construct
  source 1..20: mol_type = other RNA
caggggagggaggagcccag

SEQ ID NO: 24090 - RNA, 20 nt, synthetic construct
  source 1..20: mol_type = other RNA
aggggagggaggagcccaga

SEQ ID NO: 24091 - RNA, 20 nt, synthetic construct
  source 1..20: mol_type = other RNA
ggggagggaggagcccagag

SEQ ID NO: 24092 - RNA, 20 nt, synthetic construct
  source 1..20: mol_type = other RNA
ctctgggctcctccctcccc

SEQ ID NO: 24093 - RNA, 20 nt, synthetic construct
  source 1..20: mol_type = other RNA
cagaggggcctgcaagacac

SEQ ID NO: 24094 - RNA, 20 nt, synthetic construct
  source 1..20: mol_type = other RNA
agtgtcttgcaggcccctct

SEQ ID NO: 24095 - RNA, 20 nt, synthetic construct
  source 1..20: mol_type = other RNA
cagtgtcttgcaggcccctc

SEQ ID NO: 24096 - RNA, 20 nt, synthetic construct
  source 1..20: mol_type = other RNA
gacttcttccagtgtcttgc

SEQ ID NO: 24097 - RNA, 20 nt, synthetic construct
  source 1..20: mol_type = other RNA
actggaagaagtcagctgat

SEQ ID NO: 24098 - RNA, 20 nt, synthetic construct
  source 1..20: mol_type = other RNA
ctggaagaagtcagctgata

SEQ ID NO: 24099 - RNA, 20 nt, synthetic construct
  source 1..20: mol_type = other RNA
gaagaagtcagctgataggg

SEQ ID NO: 24100 - RNA, 20 nt, synthetic construct
  source 1..20: mol_type = other RNA
gtcagctgatagggaggtcc

SEQ ID NO: 24101 - RNA, 20 nt, synthetic construct
  source 1..20: mol_type = other RNA
tcagctgatagggaggtcct

SEQ ID NO: 24102 - RNA, 20 nt, synthetic construct
  source 1..20: mol_type = other RNA
ctgatagggaggtcctggga

SEQ ID NO: 24103 - RNA, 20 nt, synthetic construct
  source 1..20: mol_type = other RNA
tgatagggaggtcctgggat

SEQ ID NO: 24104 - RNA, 20 nt, synthetic construct
  source 1..20: mol_type = other RNA
gatagggaggtcctgggatg

SEQ ID NO: 24105 - RNA, 20 nt, synthetic construct
  source 1..20: mol_type = other RNA
gaggtcctgggatggggtcc

SEQ ID NO: 24106 - RNA, 20 nt, synthetic construct
  source 1..20: mol_type = other RNA
aggtcctgggatggggtcca

SEQ ID NO: 24107 - RNA, 20 nt, synthetic construct
  source 1..20: mol_type = other RNA
ctgggatggggtccagggcc

SEQ ID NO: 24108 - RNA, 20 nt, synthetic construct
  source 1..20: mol_type = other RNA
gatggggtccagggccaggc

SEQ ID NO: 24109 - RNA, 20 nt, synthetic construct
  source 1..20: mol_type = other RNA
atggggtccagggccaggca

SEQ ID NO: 24110 - RNA, 20 nt, synthetic construct
  source 1..20: mol_type = other RNA
gggtccagggccaggcaggg

SEQ ID NO: 24111 - RNA, 20 nt, synthetic construct
  source 1..20: mol_type = other RNA
ggtccagggccaggcaggga

SEQ ID NO: 24112 - RNA, 20 nt, synthetic construct
  source 1..20: mol_type = other RNA
agggccaggcagggagggtg

SEQ ID NO: 24113 - RNA, 20 nt, synthetic construct
  source 1..20: mol_type = other RNA
gggccaggcagggagggtga

SEQ ID NO: 24114 - RNA, 20 nt, synthetic construct
  source 1..20: mol_type = other RNA
tcaccctccctgcctggccc

SEQ ID NO: 24115 - RNA, 20 nt, synthetic construct
  source 1..20: mol_type = other RNA
aggcagggagggtgagggtg

SEQ ID NO: 24116 - RNA, 20 nt, synthetic construct
  source 1..20: mol_type = other RNA
ggcagggagggtgagggtga

SEQ ID NO: 24117 - RNA, 20 nt, synthetic construct
  source 1..20: mol_type = other RNA
gcagggagggtgagggtgag

SEQ ID NO: 24118 - RNA, 20 nt, synthetic construct
  source 1..20: mol_type = other RNA
tcaccctcaccctccctgcc

SEQ ID NO: 24119 - RNA, 20 nt, synthetic construct
  source 1..20: mol_type = other RNA
ggtgagggtgaggggagatg

SEQ ID NO: 24120 - RNA, 20 nt, synthetic construct
  source 1..20: mol_type = other RNA
ggtgaggggagatgtggtga

SEQ ID NO: 24121 - RNA, 20 nt, synthetic construct
  source 1..20: mol_type = other RNA
gtgaggggagatgtggtgac

SEQ ID NO: 24122 - RNA, 20 nt, synthetic construct
  source 1..20: mol_type = other RNA
ggagatgtggtgacgggaga

SEQ ID NO: 24123 - RNA, 20 nt, synthetic construct
  source 1..20: mol_type = other RNA
gagatgtggtgacgggagat

SEQ ID NO: 24124 - RNA, 20 nt, synthetic construct
  source 1..20: mol_type = other RNA
agatgtggtgacgggagatg

SEQ ID NO: 24125 - RNA, 20 nt, synthetic construct
  source 1..20: mol_type = other RNA
tggtgacgggagatggggtg

SEQ ID NO: 24126 - RNA, 20 nt, synthetic construct
  source 1..20: mol_type = other RNA
ggtgacgggagatggggtgt

SEQ ID NO: 24127 - RNA, 20 nt, synthetic construct
  source 1..20: mol_type = other RNA
cctcagattcttccctctcc

SEQ ID NO: 24128 - RNA, 20 nt, synthetic construct
  source 1..20: mol_type = other RNA
ctcagattcttccctctcct

SEQ ID NO: 24129 - RNA, 20 nt, synthetic construct
  source 1..20: mol_type = other RNA
ccaggagagggaagaatctg

SEQ ID NO: 24130 - RNA, 20 nt, synthetic construct
  source 1..20: mol_type = other RNA
ttcttccctctcctgggtcc

SEQ ID NO: 24131 - RNA, 20 nt, synthetic construct
  source 1..20: mol_type = other RNA
ggagtccaggacccaggaga

SEQ ID NO: 24132 - RNA, 20 nt, synthetic construct
  source 1..20: mol_type = other RNA
aggagtccaggacccaggag

SEQ ID NO: 24133 - RNA, 20 nt, synthetic construct
  source 1..20: mol_type = other RNA
atctcaggagtccaggaccc

SEQ ID NO: 24134 - RNA, 20 nt, synthetic construct
  source 1..20: mol_type = other RNA
agggttgatctcaggagtcc

SEQ ID NO: 24135 - RNA, 20 nt, synthetic construct
  source 1..20: mol_type = other RNA
agatcaacccttgagctgca

SEQ ID NO: 24136 - RNA, 20 nt, synthetic construct
  source 1..20: mol_type = other RNA
gcagctcaagggttgatctc

SEQ ID NO: 24137 - RNA, 20 nt, synthetic construct
  source 1..20: mol_type = other RNA
tgagctgcaaggctgagaag

SEQ ID NO: 24138 - RNA, 20 nt, synthetic construct
  source 1..20: mol_type = other RNA
ttctcagccttgcagctcaa

SEQ ID NO: 24139 - RNA, 20 nt, synthetic construct
  source 1..20: mol_type = other RNA
cttctcagccttgcagctca

SEQ ID NO: 24140 - RNA, 20 nt, synthetic construct
  source 1..20: mol_type = other RNA
gctgcaaggctgagaagagg

SEQ ID NO: 24141 - RNA, 20 nt, synthetic construct
  source 1..20: mol_type = other RNA
ctgcaaggctgagaagaggt

SEQ ID NO: 24142 - RNA, 20 nt, synthetic construct
  source 1..20: mol_type = other RNA
tgcaaggctgagaagaggtg

SEQ ID NO: 24143 - RNA, 20 nt, synthetic construct
  source 1..20: mol_type = other RNA
aaggctgagaagaggtgggg

SEQ ID NO: 24144 - RNA, 20 nt, synthetic construct
  source 1..20: mol_type = other RNA
aggctgagaagaggtggggt

SEQ ID NO: 24145 - RNA, 20 nt, synthetic construct
  source 1..20: mol_type = other RNA
ctgagaagaggtggggtggg

SEQ ID NO: 24146 - RNA, 20 nt, synthetic construct
  source 1..20: mol_type = other RNA
ggtgggaggagccgcagagc

SEQ ID NO: 24147 - RNA, 20 nt, synthetic construct
  source 1..20: mol_type = other RNA
gtgggaggagccgcagagca

SEQ ID NO: 24148 - RNA, 20 nt, synthetic construct
  source 1..20: mol_type = other RNA
aggagccgcagagcagggaa

SEQ ID NO: 24149 - RNA, 20 nt, synthetic construct
  source 1..20: mol_type = other RNA
ggagccgcagagcagggaat

SEQ ID NO: 24150 - RNA, 20 nt, synthetic construct
  source 1..20: mol_type = other RNA
aaagcccattccctgctctg

SEQ ID NO: 24151 - RNA, 20 nt, synthetic construct
  source 1..20: mol_type = other RNA
tgggctttcagaacccagag

SEQ ID NO: 24152 - RNA, 20 nt, synthetic construct
  source 1..20: mol_type = other RNA
cagaacccagagtggagccc

SEQ ID NO: 24153 - RNA, 20 nt, synthetic construct
  source 1..20: mol_type = other RNA
agaacccagagtggagcccc

SEQ ID NO: 24154 - RNA, 20 nt, synthetic construct
  source 1..20: mol_type = other RNA
agagtggagccccgggctgc

SEQ ID NO: 24155 - RNA, 20 nt, synthetic construct
  source 1..20: mol_type = other RNA
gcagcccggggctccactct

SEQ ID NO: 24156 - RNA, 20 nt, synthetic construct
  source 1..20: mol_type = other RNA
agcagcccggggctccactc

SEQ ID NO: 24157 - RNA, 20 nt, synthetic construct
  source 1..20: mol_type = other RNA
gccccgggctgctggctccc

SEQ ID NO: 24158 - RNA, 20 nt, synthetic construct
  source 1..20: mol_type = other RNA
acctgggagccagcagcccg

SEQ ID NO: 24159 - RNA, 20 nt, synthetic construct
  source 1..20: mol_type = other RNA
aacctgggagccagcagccc

SEQ ID NO: 24160 - RNA, 20 nt, synthetic construct
  source 1..20: mol_type = other RNA
aaacctgggagccagcagcc

SEQ ID NO: 24161 - RNA, 20 nt, synthetic construct
  source 1..20: mol_type = other RNA
aggtttcttcagacctctcc

SEQ ID NO: 24162 - RNA, 20 nt, synthetic construct
  source 1..20: mol_type = other RNA
ggagaggtctgaagaaacct

SEQ ID NO: 24163 - RNA, 20 nt, synthetic construct
  source 1..20: mol_type = other RNA
tggagaggtctgaagaaacc

SEQ ID NO: 24164 - RNA, 20 nt, synthetic construct
  source 1..20: mol_type = other RNA
cttcagacctctccaggccc

SEQ ID NO: 24165 - RNA, 20 nt, synthetic construct
  source 1..20: mol_type = other RNA
ttcagacctctccaggccct

SEQ ID NO: 24166 - RNA, 20 nt, synthetic construct
  source 1..20: mol_type = other RNA
tcagacctctccaggccctg

SEQ ID NO: 24167 - RNA, 20 nt, synthetic construct
  source 1..20: mol_type = other RNA
tggtgccccagggcctggag

SEQ ID NO: 24168 - RNA, 20 nt, synthetic construct
  source 1..20: mol_type = other RNA
ctggctggtgccccagggcc

SEQ ID NO: 24169 - RNA, 20 nt, synthetic construct
  source 1..20: mol_type = other RNA
tcttgctggctggtgcccca

SEQ ID NO: 24170 - RNA, 20 nt, synthetic construct
  source 1..20: mol_type = other RNA
ttcttgctggctggtgcccc

SEQ ID NO: 24171 - RNA, 20 nt, synthetic construct
  source 1..20: mol_type = other RNA
taggcgctgttcttgctggc

SEQ ID NO: 24172 - RNA, 20 nt, synthetic construct
  source 1..20: mol_type = other RNA
tgactaggcgctgttcttgc

SEQ ID NO: 24173 - RNA, 20 nt, synthetic construct
  source 1..20: mol_type = other RNA
agcgcctagtcaacaagagc

SEQ ID NO: 24174 - RNA, 20 nt, synthetic construct
  source 1..20: mol_type = other RNA
cctagtcaacaagagcagga

SEQ ID NO: 24175 - RNA, 20 nt, synthetic construct
  source 1..20: mol_type = other RNA
ccttcctgctcttgttgact

SEQ ID NO: 24176 - RNA, 20 nt, synthetic construct
  source 1..20: mol_type = other RNA
aggaaggaaacgtcacccag

SEQ ID NO: 24177 - RNA, 20 nt, synthetic construct
  source 1..20: mol_type = other RNA
tcacccagaggaaacccaca

SEQ ID NO: 24178 - RNA, 20 nt, synthetic construct
  source 1..20: mol_type = other RNA
cacccagaggaaacccacaa

SEQ ID NO: 24179 - RNA, 20 nt, synthetic construct
  source 1..20: mol_type = other RNA
acccagaggaaacccacaag

SEQ ID NO: 24180 - RNA, 20 nt, synthetic construct
  source 1..20: mol_type = other RNA
gaggaaacccacaaggggcg

SEQ ID NO: 24181 - RNA, 20 nt, synthetic construct
  source 1..20: mol_type = other RNA
gccccttgtgggtttcctct

SEQ ID NO: 24182 - RNA, 20 nt, synthetic construct
  source 1..20: mol_type = other RNA
cgccccttgtgggtttcctc

SEQ ID NO: 24183 - RNA, 20 nt, synthetic construct
  source 1..20: mol_type = other RNA
aacccacaaggggcgtggcc

SEQ ID NO: 24184 - RNA, 20 nt, synthetic construct
  source 1..20: mol_type = other RNA
acccacaaggggcgtggcca

SEQ ID NO: 24185 - RNA, 20 nt, synthetic construct
  source 1..20: mol_type = other RNA
cccacaaggggcgtggccag

SEQ ID NO: 24186 - RNA, 20 nt, synthetic construct
  source 1..20: mol_type = other RNA
ccacaaggggcgtggccagg

SEQ ID NO: 24187 - RNA, 20 nt, synthetic construct
  source 1..20: mol_type = other RNA
cccctggccacgccccttgt

SEQ ID NO: 24188 - RNA, 20 nt, synthetic construct
  source 1..20: mol_type = other RNA
ccccctggccacgccccttg

SEQ ID NO: 24189 - RNA, 20 nt, synthetic construct
  source 1..20: mol_type = other RNA
ccagggggtaggatcaaacc

SEQ ID NO: 24190 - RNA, 20 nt, synthetic construct
  source 1..20: mol_type = other RNA
cctggtttgatcctaccccc

SEQ ID NO: 24191 - RNA, 20 nt, synthetic construct
  source 1..20: mol_type = other RNA
ggtaggatcaaaccaggcct

SEQ ID NO: 24192 - RNA, 20 nt, synthetic construct
  source 1..20: mol_type = other RNA
ggatcaaaccaggcctgggt

SEQ ID NO: 24193 - RNA, 20 nt, synthetic construct
  source 1..20: mol_type = other RNA
gagtctggcctacccaggcc

SEQ ID NO: 24194 - RNA, 20 nt, synthetic construct
  source 1..20: mol_type = other RNA
actctgagtctggcctaccc

SEQ ID NO: 24195 - RNA, 20 nt, synthetic construct
  source 1..20: mol_type = other RNA
tgaatctgtgactctgagtc

SEQ ID NO: 24196 - RNA, 20 nt, synthetic construct
  source 1..20: mol_type = other RNA
tcagagtcacagattcagat

SEQ ID NO: 24197 - RNA, 20 nt, synthetic construct
  source 1..20: mol_type = other RNA
acagattcagatgggccaca

SEQ ID NO: 24198 - RNA, 20 nt, synthetic construct
  source 1..20: mol_type = other RNA
atgggccacatggcatctat

SEQ ID NO: 24199 - RNA, 20 nt, synthetic construct
  source 1..20: mol_type = other RNA
ggccacatggcatctatagg

SEQ ID NO: 24200 - RNA, 20 nt, synthetic construct
  source 1..20: mol_type = other RNA
atggcatctataggcggacc

SEQ ID NO: 24201 - RNA, 20 nt, synthetic construct
  source 1..20: mol_type = other RNA
gtccgcctatagatgccatg

SEQ ID NO: 24202 - RNA, 20 nt, synthetic construct
  source 1..20: mol_type = other RNA
tataggcggaccaggagcac

SEQ ID NO: 24203 - RNA, 20 nt, synthetic construct
  source 1..20: mol_type = other RNA
ctggtctgggcctgtgctcc

SEQ ID NO: 24204 - RNA, 20 nt, synthetic construct
  source 1..20: mol_type = other RNA
agaccagctgacgctgcagc

SEQ ID NO: 24205 - RNA, 20 nt, synthetic construct
  source 1..20: mol_type = other RNA
gctgcagcgtcagctggtct

SEQ ID NO: 24206 - RNA, 20 nt, synthetic construct
  source 1..20: mol_type = other RNA
tgctgcagcgtcagctggtc

SEQ ID NO: 24207 - RNA, 20 nt, synthetic construct
  source 1..20: mol_type = other RNA
gctgacgctgcagcaggtac

SEQ ID NO: 24208 - RNA, 20 nt, synthetic construct
  source 1..20: mol_type = other RNA
gtacctgctgcagcgtcagc

SEQ ID NO: 24209 - RNA, 20 nt, synthetic construct
  source 1..20: mol_type = other RNA
gtacaggcccatactaaaca

SEQ ID NO: 24210 - RNA, 20 nt, synthetic construct
  source 1..20: mol_type = other RNA
gcacacaccgtgtttagtat

SEQ ID NO: 24211 - RNA, 20 nt, synthetic construct
  source 1..20: mol_type = other RNA
tgcacacaccgtgtttagta

SEQ ID NO: 24212 - RNA, 20 nt, synthetic construct
  source 1..20: mol_type = other RNA
acggtgtgtgcacctccaca

SEQ ID NO: 24213 - RNA, 20 nt, synthetic construct
  source 1..20: mol_type = other RNA
cggtgtgtgcacctccacat

SEQ ID NO: 24214 - RNA, 20 nt, synthetic construct
  source 1..20: mol_type = other RNA
ctggcggagtgcccatgtgg

SEQ ID NO: 24215 - RNA, 20 nt, synthetic construct
  source 1..20: mol_type = other RNA
gggctggcggagtgcccatg

SEQ ID NO: 24216 - RNA, 20 nt, synthetic construct
  source 1..20: mol_type = other RNA
ggctctagatgatgggctgg

SEQ ID NO: 24217 - RNA, 20 nt, synthetic construct
  source 1..20: mol_type = other RNA
acaggctctagatgatgggc

SEQ ID NO: 24218 - RNA, 20 nt, synthetic construct
  source 1..20: mol_type = other RNA
gcagacaggctctagatgat

SEQ ID NO: 24219 - RNA, 20 nt, synthetic construct
  source 1..20: mol_type = other RNA
tgcagacaggctctagatga

SEQ ID NO: 24220 - RNA, 20 nt, synthetic construct
  source 1..20: mol_type = other RNA
tagagcctgtctgcagagcc

SEQ ID NO: 24221 - RNA, 20 nt, synthetic construct
  source 1..20: mol_type = other RNA
tgcatcctggctctgcagac

SEQ ID NO: 24222 - RNA, 20 nt, synthetic construct
  source 1..20: mol_type = other RNA
tgctcggagagtctgcatcc

SEQ ID NO: 24223 - RNA, 20 nt, synthetic construct
  source 1..20: mol_type = other RNA
agcagttgtgtctgcagccc

SEQ ID NO: 24224 - RNA, 20 nt, synthetic construct
  source 1..20: mol_type = other RNA
gggctgcagacacaactgct

SEQ ID NO: 24225 - RNA, 20 nt, synthetic construct
  source 1..20: mol_type = other RNA
cagcccaggcccagcctctc

SEQ ID NO: 24226 - RNA, 20 nt, synthetic construct
  source 1..20: mol_type = other RNA
ccaggcccagcctctcagga

SEQ ID NO: 24227 - RNA, 20 nt, synthetic construct
  source 1..20: mol_type = other RNA
caggcccagcctctcaggat

SEQ ID NO: 24228 - RNA, 20 nt, synthetic construct
  source 1..20: mol_type = other RNA
gcccagcctctcaggatggg

SEQ ID NO: 24229 - RNA, 20 nt, synthetic construct
  source 1..20: mol_type = other RNA
ccatcctgagaggctgggcc

SEQ ID NO: 24230 - RNA, 20 nt, synthetic construct
  source 1..20: mol_type = other RNA
ccagcctctcaggatgggtg

SEQ ID NO: 24231 - RNA, 20 nt, synthetic construct
  source 1..20: mol_type = other RNA
cccacccatcctgagaggct

SEQ ID NO: 24232 - RNA, 20 nt, synthetic construct
  source 1..20: mol_type = other RNA
ccccacccatcctgagaggc

SEQ ID NO: 24233 - RNA, 20 nt, synthetic construct
  source 1..20: mol_type = other RNA
ggggccccacccatcctgag

SEQ ID NO: 24234 - RNA, 20 nt, synthetic construct
  source 1..20: mol_type = other RNA
tggggccccctgtgtctgcc

SEQ ID NO: 24235 - RNA, 20 nt, synthetic construct
  source 1..20: mol_type = other RNA
ggggccccctgtgtctgccc

SEQ ID NO: 24236 - RNA, 20 nt, synthetic construct
  source 1..20: mol_type = other RNA
gctgcccgggcagacacagg

SEQ ID NO: 24237 - RNA, 20 nt, synthetic construct
  source 1..20: mol_type = other RNA
agctgcccgggcagacacag

SEQ ID NO: 24238 - RNA, 20 nt, synthetic construct
  source 1..20: mol_type = other RNA
gagctgcccgggcagacaca

SEQ ID NO: 24239 - RNA, 20 nt, synthetic construct
  source 1..20: mol_type = other RNA
ggagctgcccgggcagacac

SEQ ID NO: 24240 - RNA, 20 nt, synthetic construct
  source 1..20: mol_type = other RNA
ctgcccgggcagctccttat

SEQ ID NO: 24241 - RNA, 20 nt, synthetic construct
  source 1..20: mol_type = other RNA
tgcccgggcagctccttatt

SEQ ID NO: 24242 - RNA, 20 nt, synthetic construct
  source 1..20: mol_type = other RNA
ttcccaataaggagctgccc

SEQ ID NO: 24243 - RNA, 20 nt, synthetic construct
  source 1..20: mol_type = other RNA
tttcccaataaggagctgcc

SEQ ID NO: 24244 - RNA, 20 nt, synthetic construct
  source 1..20: mol_type = other RNA
ttattgggaaacattagaac

SEQ ID NO: 24245 - RNA, 20 nt, synthetic construct
  source 1..20: mol_type = other RNA
tattgggaaacattagaact

SEQ ID NO: 24246 - RNA, 20 nt, synthetic construct
  source 1..20: mol_type = other RNA
agttctaatgtttcccaata

SEQ ID NO: 24247 - RNA, 20 nt, synthetic construct
  source 1..20: mol_type = other RNA
ggaaacattagaactgggcc

SEQ ID NO: 24248 - RNA, 20 nt, synthetic construct
  source 1..20: mol_type = other RNA
gaaacattagaactgggcca

SEQ ID NO: 24249 - RNA, 20 nt, synthetic construct
  source 1..20: mol_type = other RNA
aggctgggaaaaatgctccc

SEQ ID NO: 24250 - RNA, 20 nt, synthetic construct
  source 1..20: mol_type = other RNA
gcatttttcccagcctctca

SEQ ID NO: 24251 - RNA, 20 nt, synthetic construct
  source 1..20: mol_type = other RNA
ttcccagcctctcatggttt

SEQ ID NO: 24252 - RNA, 20 nt, synthetic construct
  source 1..20: mol_type = other RNA
tcccagcctctcatggtttt

SEQ ID NO: 24253 - RNA, 20 nt, synthetic construct
  source 1..20: mol_type = other RNA
tcccaaaaccatgagaggct

SEQ ID NO: 24254 - RNA, 20 nt, synthetic construct
  source 1..20: mol_type = other RNA
ctcccaaaaccatgagaggc

SEQ ID NO: 24255 - RNA, 20 nt, synthetic construct
  source 1..20: mol_type = other RNA
gaagctcccaaaaccatgag

SEQ ID NO: 24256 - RNA, 20 nt, synthetic construct
  source 1..20: mol_type = other RNA
gcatgtcctgccatgctacc

SEQ ID NO: 24257 - RNA, 20 nt, synthetic construct
  source 1..20: mol_type = other RNA
catgtcctgccatgctacca

SEQ ID NO: 24258 - RNA, 20 nt, synthetic construct
  source 1..20: mol_type = other RNA
atgtcctgccatgctaccag

SEQ ID NO: 24259 - RNA, 20 nt, synthetic construct
  source 1..20: mol_type = other RNA
agtgcccctggtagcatggc

SEQ ID NO: 24260 - RNA, 20 nt, synthetic construct
  source 1..20: mol_type = other RNA
ctttagtgcccctggtagca

SEQ ID NO: 24261 - RNA, 20 nt, synthetic construct
  source 1..20: mol_type = other RNA
ggcactaaagcatgtgtccc

SEQ ID NO: 24262 - RNA, 20 nt, synthetic construct
  source 1..20: mol_type = other RNA
aaagcatgtgtcccaggccc

SEQ ID NO: 24263 - RNA, 20 nt, synthetic construct
  source 1..20: mol_type = other RNA
aagcatgtgtcccaggccca

SEQ ID NO: 24264 - RNA, 20 nt, synthetic construct
  source 1..20: mol_type = other RNA
agcatgtgtcccaggcccag

SEQ ID NO: 24265 - RNA, 20 nt, synthetic construct
  source 1..20: mol_type = other RNA
gcatgtgtcccaggcccagg

SEQ ID NO: 24266 - RNA, 20 nt, synthetic construct
  source 1..20: mol_type = other RNA
gcaaacagccccctgggcct

SEQ ID NO: 24267 - RNA, 20 nt, synthetic construct
  source 1..20: mol_type = other RNA
ggcaaacagccccctgggcc

SEQ ID NO: 24268 - RNA, 20 nt, synthetic construct
  source 1..20: mol_type = other RNA
ccagggggctgtttgccttc

SEQ ID NO: 24269 - RNA, 20 nt, synthetic construct
  source 1..20: mol_type = other RNA
cagggggctgtttgccttct

SEQ ID NO: 24270 - RNA, 20 nt, synthetic construct
  source 1..20: mol_type = other RNA
cagaaggcaaacagccccct

SEQ ID NO: 24271 - RNA, 20 nt, synthetic construct
  source 1..20: mol_type = other RNA
ccagaaggcaaacagccccc

SEQ ID NO: 24272 - RNA, 20 nt, synthetic construct
  source 1..20: mol_type = other RNA
tgggcagcccagcacttagc

SEQ ID NO: 24273 - RNA, 20 nt, synthetic construct
  source 1..20: mol_type = other RNA
atgttcaccagctaagtgct

SEQ ID NO: 24274 - RNA, 20 nt, synthetic construct
  source 1..20: mol_type = other RNA
aatgttcaccagctaagtgc

SEQ ID NO: 24275 - RNA, 20 nt, synthetic construct
  source 1..20: mol_type = other RNA
ggggctgttctgctttcagg

SEQ ID NO: 24276 - RNA, 20 nt, synthetic construct
  source 1..20: mol_type = other RNA
gaaggggctgttctgctttc

SEQ ID NO: 24277 - RNA, 20 nt, synthetic construct
  source 1..20: mol_type = other RNA
ccttcctcattcctgcaagc

SEQ ID NO: 24278 - RNA, 20 nt, synthetic construct
  source 1..20: mol_type = other RNA
tgcttgcaggaatgaggaag

SEQ ID NO: 24279 - RNA, 20 nt, synthetic construct
  source 1..20: mol_type = other RNA
ctgcttgcaggaatgaggaa

SEQ ID NO: 24280 - RNA, 20 nt, synthetic construct
  source 1..20: mol_type = other RNA
cctgcttgcaggaatgagga

SEQ ID NO: 24281 - RNA, 20 nt, synthetic construct
  source 1..20: mol_type = other RNA
tcattcctgcaagcaggcct

SEQ ID NO: 24282 - RNA, 20 nt, synthetic construct
  source 1..20: mol_type = other RNA
cattcctgcaagcaggcctc

SEQ ID NO: 24283 - RNA, 20 nt, synthetic construct
  source 1..20: mol_type = other RNA
attcctgcaagcaggcctcg

SEQ ID NO: 24284 - RNA, 20 nt, synthetic construct
  source 1..20: mol_type = other RNA
gaggcctgcttgcaggaatg

SEQ ID NO: 24285 - RNA, 20 nt, synthetic construct
  source 1..20: mol_type = other RNA
caagcaggcctcggggagcc

SEQ ID NO: 24286 - RNA, 20 nt, synthetic construct
  source 1..20: mol_type = other RNA
gctccccgaggcctgcttgc

SEQ ID NO: 24287 - RNA, 20 nt, synthetic construct
  source 1..20: mol_type = other RNA
agcaggcctcggggagccag

SEQ ID NO: 24288 - RNA, 20 nt, synthetic construct
  source 1..20: mol_type = other RNA
agtctgcccctggctccccg

SEQ ID NO: 24289 - RNA, 20 nt, synthetic construct
  source 1..20: mol_type = other RNA
ggggcagacttcctctttcg

SEQ ID NO: 24290 - RNA, 20 nt, synthetic construct
  source 1..20: mol_type = other RNA
cgaaagaggaagtctgcccc

SEQ ID NO: 24291 - RNA, 20 nt, synthetic construct
  source 1..20: mol_type = other RNA
tcttgcagattccacgaaag

SEQ ID NO: 24292 - RNA, 20 nt, synthetic construct
  source 1..20: mol_type = other RNA
tgcaagatgccaatgacttc

SEQ ID NO: 24293 - RNA, 20 nt, synthetic construct
  source 1..20: mol_type = other RNA
atgccaatgacttcaggttg

SEQ ID NO: 24294 - RNA, 20 nt, synthetic construct
  source 1..20: mol_type = other RNA
attcctcaacctgaagtcat

SEQ ID NO: 24295 - RNA, 20 nt, synthetic construct
  source 1..20: mol_type = other RNA
tgttacatcagcaaatgagt

SEQ ID NO: 24296 - RNA, 20 nt, synthetic construct
  source 1..20: mol_type = other RNA
tgctgatgtaacacaccacc

SEQ ID NO: 24297 - RNA, 20 nt, synthetic construct
  source 1..20: mol_type = other RNA
aacacaccaccaggaatttc

SEQ ID NO: 24298 - RNA, 20 nt, synthetic construct
  source 1..20: mol_type = other RNA
aggaatttctggagatgctt

SEQ ID NO: 24299 - RNA, 20 nt, synthetic construct
  source 1..20: mol_type = other RNA
aaagcatctccagaaattcc

SEQ ID NO: 24300 - RNA, 20 nt, synthetic construct
  source 1..20: mol_type = other RNA
ggagatgctttggtttcact

SEQ ID NO: 24301 - RNA, 20 nt, synthetic construct
  source 1..20: mol_type = other RNA
tgctttggtttcacttggac

SEQ ID NO: 24302 - RNA, 20 nt, synthetic construct
  source 1..20: mol_type = other RNA
cacttggactggcagagccc

SEQ ID NO: 24303 - RNA, 20 nt, synthetic construct
  source 1..20: mol_type = other RNA
agagcccaggcttcaaccca

SEQ ID NO: 24304 - RNA, 20 nt, synthetic construct
  source 1..20: mol_type = other RNA
gcttcaacccacggcttgct

SEQ ID NO: 24305 - RNA, 20 nt, synthetic construct
  source 1..20: mol_type = other RNA
gcaagccgtgggttgaagcc

SEQ ID NO: 24306 - RNA, 20 nt, synthetic construct
  source 1..20: mol_type = other RNA
acccacggcttgcttggaca

SEQ ID NO: 24307 - RNA, 20 nt, synthetic construct
  source 1..20: mol_type = other RNA
tccttgtccaagcaagccgt

SEQ ID NO: 24308 - RNA, 20 nt, synthetic construct
  source 1..20: mol_type = other RNA
gtccttgtccaagcaagccg

SEQ ID NO: 24309 - RNA, 20 nt, synthetic construct
  source 1..20: mol_type = other RNA
agaaataaatcaggcacata

SEQ ID NO: 24310 - RNA, 20 nt, synthetic construct
  source 1..20: mol_type = other RNA
gaggctcaaagaaataaatc

SEQ ID NO: 24311 - RNA, 20 nt, synthetic construct
  source 1..20: mol_type = other RNA
cagtttgcccatctattaaa

SEQ ID NO: 24312 - RNA, 20 nt, synthetic construct
  source 1..20: mol_type = other RNA
agtttgcccatctattaaat

SEQ ID NO: 24313 - RNA, 20 nt, synthetic construct
  source 1..20: mol_type = other RNA
tttaatagatgggcaaactg

SEQ ID NO: 24314 - RNA, 20 nt, synthetic construct
  source 1..20: mol_type = other RNA
tctattaaatgggacatcat

SEQ ID NO: 24315 - RNA, 20 nt, synthetic construct
  source 1..20: mol_type = other RNA
tgatgtcccatttaatagat

SEQ ID NO: 24316 - RNA, 20 nt, synthetic construct
  source 1..20: mol_type = other RNA
atgatgtcccatttaataga

SEQ ID NO: 24317 - RNA, 20 nt, synthetic construct
  source 1..20: mol_type = other RNA
gacatcataggtttaccaag

SEQ ID NO: 24318 - RNA, 20 nt, synthetic construct
  source 1..20: mol_type = other RNA
agaggcttcaattcagcaaa

SEQ ID NO: 24319 - RNA, 20 nt, synthetic construct
  source 1..20: mol_type = other RNA
tttgctgaattgaagcctct

SEQ ID NO: 24320 - RNA, 20 nt, synthetic construct
  source 1..20: mol_type = other RNA
agagtctctctctctttccc

SEQ ID NO: 24321 - RNA, 20 nt, synthetic construct
  source 1..20: mol_type = other RNA
tctctctctctttcccaggc

SEQ ID NO: 24322 - RNA, 20 nt, synthetic construct
  source 1..20: mol_type = other RNA
tttcccaggctggagtgcag

SEQ ID NO: 24323 - RNA, 20 nt, synthetic construct
  source 1..20: mol_type = other RNA
ttgccactgcactccagcct

SEQ ID NO: 24324 - RNA, 20 nt, synthetic construct
  source 1..20: mol_type = other RNA
cttgccactgcactccagcc

SEQ ID NO: 24325 - RNA, 20 nt, synthetic construct
  source 1..20: mol_type = other RNA
ggagtgcagtggcaagatct

SEQ ID NO: 24326 - RNA, 20 nt, synthetic construct
  source 1..20: mol_type = other RNA
tgcaagctccctccacctcc

SEQ ID NO: 24327 - RNA, 20 nt, synthetic construct
  source 1..20: mol_type = other RNA
gcaagctccctccacctcct

SEQ ID NO: 24328 - RNA, 20 nt, synthetic construct
  source 1..20: mol_type = other RNA
gctggaacccaggaggtgga

SEQ ID NO: 24329 - RNA, 20 nt, synthetic construct
  source 1..20: mol_type = other RNA
cgctggaacccaggaggtgg

SEQ ID NO: 24330 - RNA, 20 nt, synthetic construct
  source 1..20: mol_type = other RNA
aatcgctggaacccaggagg

SEQ ID NO: 24331 - RNA, 20 nt, synthetic construct
  source 1..20: mol_type = other RNA
gagaatcgctggaacccagg

SEQ ID NO: 24332 - RNA, 20 nt, synthetic construct
  source 1..20: mol_type = other RNA
caggagaatcgctggaaccc

SEQ ID NO: 24333 - RNA, 20 nt, synthetic construct
  source 1..20: mol_type = other RNA
ggctgatgcaggagaatcgc

SEQ ID NO: 24334 - RNA, 20 nt, synthetic construct
  source 1..20: mol_type = other RNA
cctgcatcagcccagcttcc

SEQ ID NO: 24335 - RNA, 20 nt, synthetic construct
  source 1..20: mol_type = other RNA
ctgcatcagcccagcttcct

SEQ ID NO: 24336 - RNA, 20 nt, synthetic construct
  source 1..20: mol_type = other RNA
ccaggaagctgggctgatgc

SEQ ID NO: 24337 - RNA, 20 nt, synthetic construct
  source 1..20: mol_type = other RNA
agcccagcttcctgggcagt

SEQ ID NO: 24338 - RNA, 20 nt, synthetic construct
  source 1..20: mol_type = other RNA
gcccagcttcctgggcagtt

SEQ ID NO: 24339 - RNA, 20 nt, synthetic construct
  source 1..20: mol_type = other RNA
tcccaactgcccaggaagct

SEQ ID NO: 24340 - RNA, 20 nt, synthetic construct
  source 1..20: mol_type = other RNA
atcccaactgcccaggaagc

SEQ ID NO: 24341 - RNA, 20 nt, synthetic construct
  source 1..20: mol_type = other RNA
gactgtaatcccaactgccc

SEQ ID NO: 24342 - RNA, 20 nt, synthetic construct
  source 1..20: mol_type = other RNA
cagtcactcaccaccacgcc

SEQ ID NO: 24343 - RNA, 20 nt, synthetic construct
  source 1..20: mol_type = other RNA
aaacaattagccaggcgtgg

SEQ ID NO: 24344 - RNA, 20 nt, synthetic construct
  source 1..20: mol_type = other RNA
acaaaacaattagccaggcg

SEQ ID NO: 24345 - RNA, 20 nt, synthetic construct
  source 1..20: mol_type = other RNA
aaaatacaaaacaattagcc

SEQ ID NO: 24346 - RNA, 20 nt, synthetic construct
  source 1..20: mol_type = other RNA
ttttgtatttttagtagaga

SEQ ID NO: 24347 - RNA, 20 nt, synthetic construct
  source 1..20: mol_type = other RNA
tttgtatttttagtagagat

SEQ ID NO: 24348 - RNA, 20 nt, synthetic construct
  source 1..20: mol_type = other RNA
ttgtatttttagtagagatg

SEQ ID NO: 24349 - RNA, 20 nt, synthetic construct
  source 1..20: mol_type = other RNA
atgttagccagtctgatccg

SEQ ID NO: 24350 - RNA, 20 nt, synthetic construct
  source 1..20: mol_type = other RNA
tcggatcagactggctaaca

SEQ ID NO: 24351 - RNA, 20 nt, synthetic construct
  source 1..20: mol_type = other RNA
cggatcacctcggatcagac

SEQ ID NO: 24352 - RNA, 20 nt, synthetic construct
  source 1..20: mol_type = other RNA
ccgaggtgatccgcccactt

SEQ ID NO: 24353 - RNA, 20 nt, synthetic construct
  source 1..20: mol_type = other RNA
ccgaagtgggcggatcacct

SEQ ID NO: 24354 - RNA, 20 nt, synthetic construct
  source 1..20: mol_type = other RNA
tttcgggaggccgaagtggg

SEQ ID NO: 24355 - RNA, 20 nt, synthetic construct
  source 1..20: mol_type = other RNA
acttcggcctcccgaaatgt

SEQ ID NO: 24356 - RNA, 20 nt, synthetic construct
  source 1..20: mol_type = other RNA
cttcggcctcccgaaatgtt

SEQ ID NO: 24357 - RNA, 20 nt, synthetic construct
  source 1..20: mol_type = other RNA
acatttcgggaggccgaagt

SEQ ID NO: 24358 - RNA, 20 nt, synthetic construct
  source 1..20: mol_type = other RNA
aacatttcgggaggccgaag

SEQ ID NO: 24359 - RNA, 20 nt, synthetic construct
  source 1..20: mol_type = other RNA
tcccgaaatgttgggattac

SEQ ID NO: 24360 - RNA, 20 nt, synthetic construct
  source 1..20: mol_type = other RNA
tgtaatcccaacatttcggg

SEQ ID NO: 24361 - RNA, 20 nt, synthetic construct
  source 1..20: mol_type = other RNA
acctgtaatcccaacatttc

SEQ ID NO: 24362 - RNA, 20 nt, synthetic construct
  source 1..20: mol_type = other RNA
cacctgtaatcccaacattt

SEQ ID NO: 24363 - RNA, 20 nt, synthetic construct
  source 1..20: mol_type = other RNA
caggtgtgagcctccgtgcc

SEQ ID NO: 24364 - RNA, 20 nt, synthetic construct
  source 1..20: mol_type = other RNA
tttatttaggccaggcacgg

SEQ ID NO: 24365 - RNA, 20 nt, synthetic construct
  source 1..20: mol_type = other RNA
aaatttatttaggccaggca

SEQ ID NO: 24366 - RNA, 20 nt, synthetic construct
  source 1..20: mol_type = other RNA
ttataaaatttatttaggcc

SEQ ID NO: 24367 - RNA, 20 nt, synthetic construct
  source 1..20: mol_type = other RNA
aacatttataaaatttattt

SEQ ID NO: 24368 - RNA, 20 nt, synthetic construct
  source 1..20: mol_type = other RNA
taaatgttagttttaaaaaa

SEQ ID NO: 24369 - RNA, 20 nt, synthetic construct
  source 1..20: mol_type = other RNA
atggctaataagcacattgt

SEQ ID NO: 24370 - RNA, 20 nt, synthetic construct
  source 1..20: mol_type = other RNA
aatatcagattgaccagaag

SEQ ID NO: 24371 - RNA, 20 nt, synthetic construct
  source 1..20: mol_type = other RNA
gcacagcacttttccacttc

SEQ ID NO: 24372 - RNA, 20 nt, synthetic construct
  source 1..20: mol_type = other RNA
gaaaagtgctgtgctaaaag

SEQ ID NO: 24373 - RNA, 20 nt, synthetic construct
  source 1..20: mol_type = other RNA
aaaagtgctgtgctaaaagt

SEQ ID NO: 24374 - RNA, 20 nt, synthetic construct
  source 1..20: mol_type = other RNA
tgtgctaaaagtgggatgat

SEQ ID NO: 24375 - RNA, 20 nt, synthetic construct
  source 1..20: mol_type = other RNA
gtgctaaaagtgggatgatc

SEQ ID NO: 24376 - RNA, 20 nt, synthetic construct
  source 1..20: mol_type = other RNA
ctaaaagtgggatgatcggg

SEQ ID NO: 24377 - RNA, 20 nt, synthetic construct
  source 1..20: mol_type = other RNA
aggctctgagcactccgtga

SEQ ID NO: 24378 - RNA, 20 nt, synthetic construct
  source 1..20: mol_type = other RNA
tggagtctcacggtccttca

SEQ ID NO: 24379 - RNA, 20 nt, synthetic construct
  source 1..20: mol_type = other RNA
gaccgtgagactccatgtag

SEQ ID NO: 24380 - RNA, 20 nt, synthetic construct
  source 1..20: mol_type = other RNA
accgtgagactccatgtagc

SEQ ID NO: 24381 - RNA, 20 nt, synthetic construct
  source 1..20: mol_type = other RNA
gtgagactccatgtagcggg

SEQ ID NO: 24382 - RNA, 20 nt, synthetic construct
  source 1..20: mol_type = other RNA
tcccgctacatggagtctca

SEQ ID NO: 24383 - RNA, 20 nt, synthetic construct
  source 1..20: mol_type = other RNA
actccatgtagcgggaggaa

SEQ ID NO: 24384 - RNA, 20 nt, synthetic construct
  source 1..20: mol_type = other RNA
atgtagcgggaggaatggcc

SEQ ID NO: 24385 - RNA, 20 nt, synthetic construct
  source 1..20: mol_type = other RNA
aggccattcctcccgctaca

SEQ ID NO: 24386 - RNA, 20 nt, synthetic construct
  source 1..20: mol_type = other RNA
cgggaggaatggcctggagg

SEQ ID NO: 24387 - RNA, 20 nt, synthetic construct
  source 1..20: mol_type = other RNA
gggaggaatggcctggagga

SEQ ID NO: 24388 - RNA, 20 nt, synthetic construct
  source 1..20: mol_type = other RNA
tggcctggaggagggctgtg

SEQ ID NO: 24389 - RNA, 20 nt, synthetic construct
  source 1..20: mol_type = other RNA
ggcctggaggagggctgtgt

SEQ ID NO: 24390 - RNA, 20 nt, synthetic construct
  source 1..20: mol_type = other RNA
agcccacacagccctcctcc

SEQ ID NO: 24391 - RNA, 20 nt, synthetic construct
  source 1..20: mol_type = other RNA
ctcctcacaccagccagttc

SEQ ID NO: 24392 - RNA, 20 nt, synthetic construct
  source 1..20: mol_type = other RNA
cagaactggctggtgtgagg

SEQ ID NO: 24393 - RNA, 20 nt, synthetic construct
  source 1..20: mol_type = other RNA
tgccagaactggctggtgtg

SEQ ID NO: 24394 - RNA, 20 nt, synthetic construct
  source 1..20: mol_type = other RNA
gagttggtgccagaactggc

SEQ ID NO: 24395 - RNA, 20 nt, synthetic construct
  source 1..20: mol_type = other RNA
tagagagttggtgccagaac

SEQ ID NO: 24396 - RNA, 20 nt, synthetic construct
  source 1..20: mol_type = other RNA
ccaactctctagacaccaac

SEQ ID NO: 24397 - RNA, 20 nt, synthetic construct
  source 1..20: mol_type = other RNA
ccagttggtgtctagagagt

SEQ ID NO: 24398 - RNA, 20 nt, synthetic construct
  source 1..20: mol_type = other RNA
ttgcactgtaggacaccagt

SEQ ID NO: 24399 - RNA, 20 nt, synthetic construct
  source 1..20: mol_type = other RNA
cagtgtcagaattgcactgt

SEQ ID NO: 24400 - RNA, 20 nt, synthetic construct
  source 1..20: mol_type = other RNA
caattctgacactgactgcc

SEQ ID NO: 24401 - RNA, 20 nt, synthetic construct
  source 1..20: mol_type = other RNA
tgacactgactgcctggagt

SEQ ID NO: 24402 - RNA, 20 nt, synthetic construct
  source 1..20: mol_type = other RNA
gagttggcatcaaacctcac

SEQ ID NO: 24403 - RNA, 20 nt, synthetic construct
  source 1..20: mol_type = other RNA
tgaggtttgatgccaactcc

SEQ ID NO: 24404 - RNA, 20 nt, synthetic construct
  source 1..20: mol_type = other RNA
gcatcaaacctcacaggttt

SEQ ID NO: 24405 - RNA, 20 nt, synthetic construct
  source 1..20: mol_type = other RNA
catcaaacctcacaggttta

SEQ ID NO: 24406 - RNA, 20 nt, synthetic construct
  source 1..20: mol_type = other RNA
actgaaaccctaaacctgtg

SEQ ID NO: 24407 - RNA, 20 nt, synthetic construct
  source 1..20: mol_type = other RNA
ttagggtttcagtgaagagc

SEQ ID NO: 24408 - RNA, 20 nt, synthetic construct
  source 1..20: mol_type = other RNA
tgcaactggcatctgatatg

SEQ ID NO: 24409 - RNA, 20 nt, synthetic construct
  source 1..20: mol_type = other RNA
atcagatgccagttgcaaat

SEQ ID NO: 24410 - RNA, 20 nt, synthetic construct
  source 1..20: mol_type = other RNA
tcagatgccagttgcaaatg

SEQ ID NO: 24411 - RNA, 20 nt, synthetic construct
  source 1..20: mol_type = other RNA
ctgggcaccccatttgcaac

SEQ ID NO: 24412 - RNA, 20 nt, synthetic construct
  source 1..20: mol_type = other RNA
aaatggggtgcccagaccac

SEQ ID NO: 24413 - RNA, 20 nt, synthetic construct
  source 1..20: mol_type = other RNA
gacagagatgccagtggtct

SEQ ID NO: 24414 - RNA, 20 nt, synthetic construct
  source 1..20: mol_type = other RNA
agacagagatgccagtggtc

SEQ ID NO: 24415 - RNA, 20 nt, synthetic construct
  source 1..20: mol_type = other RNA
aagtcagacagagatgccag

SEQ ID NO: 24416 - RNA, 20 nt, synthetic construct
  source 1..20: mol_type = other RNA
gcctcagcctcccaaagtcc

SEQ ID NO: 24417 - RNA, 20 nt, synthetic construct
  source 1..20: mol_type = other RNA
cctcagcctcccaaagtcct

SEQ ID NO: 24418 - RNA, 20 nt, synthetic construct
  source 1..20: mol_type = other RNA
tcccaaagtcctgggattac

SEQ ID NO: 24419 - RNA, 20 nt, synthetic construct
  source 1..20: mol_type = other RNA
caggcatgagccaccctgtc

SEQ ID NO: 24420 - RNA, 20 nt, synthetic construct
  source 1..20: mol_type = other RNA
aaataaaaggccagacaggg

SEQ ID NO: 24421 - RNA, 20 nt, synthetic construct
  source 1..20: mol_type = other RNA
aacaaataaaaggccagaca

SEQ ID NO: 24422 - RNA, 20 nt, synthetic construct
  source 1..20: mol_type = other RNA
aaacaaataaaaggccagac

SEQ ID NO: 24423 - RNA, 20 nt, synthetic construct
  source 1..20: mol_type = other RNA
aaaataaataaacaaataaa

SEQ ID NO: 24424 - RNA, 20 nt, synthetic construct
  source 1..20: mol_type = other RNA
tatttatttatttatttttg

SEQ ID NO: 24425 - RNA, 20 nt, synthetic construct
  source 1..20: mol_type = other RNA
agacatggagaggcattgcg

SEQ ID NO: 24426 - RNA, 20 nt, synthetic construct
  source 1..20: mol_type = other RNA
tggggtagatagacatggag

SEQ ID NO: 24427 - RNA, 20 nt, synthetic construct
  source 1..20: mol_type = other RNA
ggaactggggtagatagaca

SEQ ID NO: 24428 - RNA, 20 nt, synthetic construct
  source 1..20: mol_type = other RNA
gtgctaggagtcgggaactg

SEQ ID NO: 24429 - RNA, 20 nt, synthetic construct
  source 1..20: mol_type = other RNA
ggtgctaggagtcgggaact

SEQ ID NO: 24430 - RNA, 20 nt, synthetic construct
  source 1..20: mol_type = other RNA
tggtgctaggagtcgggaac

SEQ ID NO: 24431 - RNA, 20 nt, synthetic construct
  source 1..20: mol_type = other RNA
ccgactcctagcaccacatc

SEQ ID NO: 24432 - RNA, 20 nt, synthetic construct
  source 1..20: mol_type = other RNA
cagatgtggtgctaggagtc

SEQ ID NO: 24433 - RNA, 20 nt, synthetic construct
  source 1..20: mol_type = other RNA
ccagatgtggtgctaggagt

SEQ ID NO: 24434 - RNA, 20 nt, synthetic construct
  source 1..20: mol_type = other RNA
caccacatctggcacatcat

SEQ ID NO: 24435 - RNA, 20 nt, synthetic construct
  source 1..20: mol_type = other RNA
cacatctggcacatcatagg

SEQ ID NO: 24436 - RNA, 20 nt, synthetic construct
  source 1..20: mol_type = other RNA
cacctatgatgtgccagatg

SEQ ID NO: 24437 - RNA, 20 nt, synthetic construct
  source 1..20: mol_type = other RNA
cataggtggtcagcatttat

SEQ ID NO: 24438 - RNA, 20 nt, synthetic construct
  source 1..20: mol_type = other RNA
gcatttattggatgaatgaa

SEQ ID NO: 24439 - RNA, 20 nt, synthetic construct
  source 1..20: mol_type = other RNA
cttgaagtacgaatagaatt

SEQ ID NO: 24440 - RNA, 20 nt, synthetic construct
  source 1..20: mol_type = other RNA
acgaatagaatttggcgaag

SEQ ID NO: 24441 - RNA, 20 nt, synthetic construct
  source 1..20: mol_type = other RNA
agaatttggcgaagtggaca

SEQ ID NO: 24442 - RNA, 20 nt, synthetic construct
  source 1..20: mol_type = other RNA
tttggcgaagtggacaaggc

SEQ ID NO: 24443 - RNA, 20 nt, synthetic construct
  source 1..20: mol_type = other RNA
aaggcaggaaatgtgtattc

SEQ ID NO: 24444 - RNA, 20 nt, synthetic construct
  source 1..20: mol_type = other RNA
gaaatgtgtattcaggcatg

SEQ ID NO: 24445 - RNA, 20 nt, synthetic construct
  source 1..20: mol_type = other RNA
atgaggcttagcttgtgcat

SEQ ID NO: 24446 - RNA, 20 nt, synthetic construct
  source 1..20: mol_type = other RNA
tagcttgtgcataggtagaa

SEQ ID NO: 24447 - RNA, 20 nt, synthetic construct
  source 1..20: mol_type = other RNA
tagaaaggcatgaaaaaaca

SEQ ID NO: 24448 - RNA, 20 nt, synthetic construct
  source 1..20: mol_type = other RNA
gaatccacaaatagtaagag

SEQ ID NO: 24449 - RNA, 20 nt, synthetic construct
  source 1..20: mol_type = other RNA
aatccacaaatagtaagaga

SEQ ID NO: 24450 - RNA, 20 nt, synthetic construct
  source 1..20: mol_type = other RNA
tagccctctcttactatttg

SEQ ID NO: 24451 - RNA, 20 nt, synthetic construct
  source 1..20: mol_type = other RNA
gagagggctaagtcgttgtg

SEQ ID NO: 24452 - RNA, 20 nt, synthetic construct
  source 1..20: mol_type = other RNA
agagggctaagtcgttgtgt

SEQ ID NO: 24453 - RNA, 20 nt, synthetic construct
  source 1..20: mol_type = other RNA
gagggctaagtcgttgtgtg

SEQ ID NO: 24454 - RNA, 20 nt, synthetic construct
  source 1..20: mol_type = other RNA
agggctaagtcgttgtgtgg

SEQ ID NO: 24455 - RNA, 20 nt, synthetic construct
  source 1..20: mol_type = other RNA
taagtcgttgtgtgggggag

SEQ ID NO: 24456 - RNA, 20 nt, synthetic construct
  source 1..20: mol_type = other RNA
gaggagaaatgaagttcaaa

SEQ ID NO: 24457 - RNA, 20 nt, synthetic construct
  source 1..20: mol_type = other RNA
agaaatgaagttcaaatggt

SEQ ID NO: 24458 - RNA, 20 nt, synthetic construct
  source 1..20: mol_type = other RNA
gaagttcaaatggtaggcaa

SEQ ID NO: 24459 - RNA, 20 nt, synthetic construct
  source 1..20: mol_type = other RNA
aaatggtaggcaaaggtcag

SEQ ID NO: 24460 - RNA, 20 nt, synthetic construct
  source 1..20: mol_type = other RNA
aatggtaggcaaaggtcagt

SEQ ID NO: 24461 - RNA, 20 nt, synthetic construct
  source 1..20: mol_type = other RNA
taggcaaaggtcagtgggca

SEQ ID NO: 24462 - RNA, 20 nt, synthetic construct
  source 1..20: mol_type = other RNA
aggcaaaggtcagtgggcaa

SEQ ID NO: 24463 - RNA, 20 nt, synthetic construct
  source 1..20: mol_type = other RNA
aaattcaagtgcaatttaca

SEQ ID NO: 24464 - RNA, 20 nt, synthetic construct
  source 1..20: mol_type = other RNA
gcacttgaattttattcttt

SEQ ID NO: 24465 - RNA, 20 nt, synthetic construct
  source 1..20: mol_type = other RNA
aattttattctttaggcaaa

SEQ ID NO: 24466 - RNA, 20 nt, synthetic construct
  source 1..20: mol_type = other RNA
taggcaaaaggaagagttta

SEQ ID NO: 24467 - RNA, 20 nt, synthetic construct
  source 1..20: mol_type = other RNA
aggcaaaaggaagagtttaa

SEQ ID NO: 24468 - RNA, 20 nt, synthetic construct
  source 1..20: mol_type = other RNA
gtttaagggtttcaagaaga

SEQ ID NO: 24469 - RNA, 20 nt, synthetic construct
  source 1..20: mol_type = other RNA
aagaagaaggacacgaccag

SEQ ID NO: 24470 - RNA, 20 nt, synthetic construct
  source 1..20: mol_type = other RNA
agaagaaggacacgaccagt

SEQ ID NO: 24471 - RNA, 20 nt, synthetic construct
  source 1..20: mol_type = other RNA
ggacacgaccagtgggtttt

SEQ ID NO: 24472 - RNA, 20 nt, synthetic construct
  source 1..20: mol_type = other RNA
atgatcttcctaaaacccac

SEQ ID NO: 24473 - RNA, 20 nt, synthetic construct
  source 1..20: mol_type = other RNA
ttttaggaagatcattctga

SEQ ID NO: 24474 - RNA, 20 nt, synthetic construct
  source 1..20: mol_type = other RNA
tcattctgatggcctttcag

SEQ ID NO: 24475 - RNA, 20 nt, synthetic construct
  source 1..20: mol_type = other RNA
tctgatggcctttcagagga

SEQ ID NO: 24476 - RNA, 20 nt, synthetic construct
  source 1..20: mol_type = other RNA
ggcctttcagaggatggctg

SEQ ID NO: 24477 - RNA, 20 nt, synthetic construct
  source 1..20: mol_type = other RNA
ctcctcagccatcctctgaa

SEQ ID NO: 24478 - RNA, 20 nt, synthetic construct
  source 1..20: mol_type = other RNA
gatggctgaggagagctagc

SEQ ID NO: 24479 - RNA, 20 nt, synthetic construct
  source 1..20: mol_type = other RNA
atggctgaggagagctagca

SEQ ID NO: 24480 - RNA, 20 nt, synthetic construct
  source 1..20: mol_type = other RNA
gctgaggagagctagcaggg

SEQ ID NO: 24481 - RNA, 20 nt, synthetic construct
  source 1..20: mol_type = other RNA
aggagagctagcagggaggc

SEQ ID NO: 24482 - RNA, 20 nt, synthetic construct
  source 1..20: mol_type = other RNA
ggagagctagcagggaggca

SEQ ID NO: 24483 - RNA, 20 nt, synthetic construct
  source 1..20: mol_type = other RNA
gagctagcagggaggcaggg

SEQ ID NO: 24484 - RNA, 20 nt, synthetic construct
  source 1..20: mol_type = other RNA
ggaggcagggaggtcgagtc

SEQ ID NO: 24485 - RNA, 20 nt, synthetic construct
  source 1..20: mol_type = other RNA
gaggcagggaggtcgagtca

SEQ ID NO: 24486 - RNA, 20 nt, synthetic construct
  source 1..20: mol_type = other RNA
aggcagggaggtcgagtcag

SEQ ID NO: 24487 - RNA, 20 nt, synthetic construct
  source 1..20: mol_type = other RNA
cgagtcaggggattttgacc

SEQ ID NO: 24488 - RNA, 20 nt, synthetic construct
  source 1..20: mol_type = other RNA
caggggattttgaccaggcc

SEQ ID NO: 24489 - RNA, 20 nt, synthetic construct
  source 1..20: mol_type = other RNA
gattttgaccaggccaggtt

SEQ ID NO: 24490 - RNA, 20 nt, synthetic construct
  source 1..20: mol_type = other RNA
aggccaggttaggtgctatg

SEQ ID NO: 24491 - RNA, 20 nt, synthetic construct
  source 1..20: mol_type = other RNA
tcatagcacctaacctggcc

SEQ ID NO: 24492 - RNA, 20 nt, synthetic construct
  source 1..20: mol_type = other RNA
aggttaggtgctatgaggcc

SEQ ID NO: 24493 - RNA, 20 nt, synthetic construct
  source 1..20: mol_type = other RNA
ggttaggtgctatgaggccc

SEQ ID NO: 24494 - RNA, 20 nt, synthetic construct
  source 1..20: mol_type = other RNA
gggcctcatagcacctaacc

SEQ ID NO: 24495 - RNA, 20 nt, synthetic construct
  source 1..20: mol_type = other RNA
gtgctatgaggcccgggctt

SEQ ID NO: 24496 - RNA, 20 nt, synthetic construct
  source 1..20: mol_type = other RNA
ccgggctttggagaagaacc

SEQ ID NO: 24497 - RNA, 20 nt, synthetic construct
  source 1..20: mol_type = other RNA
ctggttcttctccaaagccc

SEQ ID NO: 24498 - RNA, 20 nt, synthetic construct
  source 1..20: mol_type = other RNA
cctggttcttctccaaagcc

SEQ ID NO: 24499 - RNA, 20 nt, synthetic construct
  source 1..20: mol_type = other RNA
tttggagaagaaccaggaaa

SEQ ID NO: 24500 - RNA, 20 nt, synthetic construct
  source 1..20: mol_type = other RNA
aagaaccaggaaatggcaac

SEQ ID NO: 24501 - RNA, 20 nt, synthetic construct
  source 1..20: mol_type = other RNA
aaccaggaaatggcaactgg

SEQ ID NO: 24502 - RNA, 20 nt, synthetic construct
  source 1..20: mol_type = other RNA
tgcctccagttgccatttcc

SEQ ID NO: 24503 - RNA, 20 nt, synthetic construct
  source 1..20: mol_type = other RNA
atggcaactggaggcaagaa

SEQ ID NO: 24504 - RNA, 20 nt, synthetic construct
  source 1..20: mol_type = other RNA
tggcaactggaggcaagaaa

SEQ ID NO: 24505 - RNA, 20 nt, synthetic construct
  source 1..20: mol_type = other RNA
ggcaactggaggcaagaaag

SEQ ID NO: 24506 - RNA, 20 nt, synthetic construct
  source 1..20: mol_type = other RNA
tggaggcaagaaaggggaga

SEQ ID NO: 24507 - RNA, 20 nt, synthetic construct
  source 1..20: mol_type = other RNA
aaggggagaaggccaaagcc

SEQ ID NO: 24508 - RNA, 20 nt, synthetic construct
  source 1..20: mol_type = other RNA
aggggagaaggccaaagcct

SEQ ID NO: 24509 - RNA, 20 nt, synthetic construct
  source 1..20: mol_type = other RNA
tgttgatggttcccaggctt

SEQ ID NO: 24510 - RNA, 20 nt, synthetic construct
  source 1..20: mol_type = other RNA
cttaagtgttgatggttccc

SEQ ID NO: 24511 - RNA, 20 nt, synthetic construct
  source 1..20: mol_type = other RNA
ttactgttcttaagtgttga

SEQ ID NO: 24512 - RNA, 20 nt, synthetic construct
  source 1..20: mol_type = other RNA
aacatctaaagagaacaaga

SEQ ID NO: 24513 - RNA, 20 nt, synthetic construct
  source 1..20: mol_type = other RNA
ctaaagagaacaagaaggaa

SEQ ID NO: 24514 - RNA, 20 nt, synthetic construct
  source 1..20: mol_type = other RNA
aagaaggaatggccagaaga

SEQ ID NO: 24515 - RNA, 20 nt, synthetic construct
  source 1..20: mol_type = other RNA
atggccagaagaaggaaaac

SEQ ID NO: 24516 - RNA, 20 nt, synthetic construct
  source 1..20: mol_type = other RNA
ctttcctgttttccttcttc

SEQ ID NO: 24517 - RNA, 20 nt, synthetic construct
  source 1..20: mol_type = other RNA
aggaaaacaggaaagaactg

SEQ ID NO: 24518 - RNA, 20 nt, synthetic construct
  source 1..20: mol_type = other RNA
aacaggaaagaactgaggcg

SEQ ID NO: 24519 - RNA, 20 nt, synthetic construct
  source 1..20: mol_type = other RNA
acaggaaagaactgaggcgt

SEQ ID NO: 24520 - RNA, 20 nt, synthetic construct
  source 1..20: mol_type = other RNA
tgggagcgcaagagagagaa

SEQ ID NO: 24521 - RNA, 20 nt, synthetic construct
  source 1..20: mol_type = other RNA
agagagagaatggttcgaga

SEQ ID NO: 24522 - RNA, 20 nt, synthetic construct
  source 1..20: mol_type = other RNA
ttcgagaaggaagcagtcac

SEQ ID NO: 24523 - RNA, 20 nt, synthetic construct
  source 1..20: mol_type = other RNA
ggaagcagtcacaggtgtca

SEQ ID NO: 24524 - RNA, 20 nt, synthetic construct
  source 1..20: mol_type = other RNA
gtcacaggtgtcaaggccat

SEQ ID NO: 24525 - RNA, 20 nt, synthetic construct
  source 1..20: mol_type = other RNA
tcacaggtgtcaaggccatt

SEQ ID NO: 24526 - RNA, 20 nt, synthetic construct
  source 1..20: mol_type = other RNA
caggtgtcaaggccattggg

SEQ ID NO: 24527 - RNA, 20 nt, synthetic construct
  source 1..20: mol_type = other RNA
ttgggaggtcaagtgagata

SEQ ID NO: 24528 - RNA, 20 nt, synthetic construct
  source 1..20: mol_type = other RNA
tatctcacttgacctcccaa

SEQ ID NO: 24529 - RNA, 20 nt, synthetic construct
  source 1..20: mol_type = other RNA
tcaagtgagataaggactga

SEQ ID NO: 24530 - RNA, 20 nt, synthetic construct
  source 1..20: mol_type = other RNA
ggactgaaggtcccaccaat

SEQ ID NO: 24531 - RNA, 20 nt, synthetic construct
  source 1..20: mol_type = other RNA
gactgaaggtcccaccaatt

SEQ ID NO: 24532 - RNA, 20 nt, synthetic construct
  source 1..20: mol_type = other RNA
gtcccaccaattgggccatc

SEQ ID NO: 24533 - RNA, 20 nt, synthetic construct
  source 1..20: mol_type = other RNA
ctcctgatggcccaattggt

SEQ ID NO: 24534 - RNA, 20 nt, synthetic construct
  source 1..20: mol_type = other RNA
gctcctgatggcccaattgg

SEQ ID NO: 24535 - RNA, 20 nt, synthetic construct
  source 1..20: mol_type = other RNA
tgtgctcctgatggcccaat

SEQ ID NO: 24536 - RNA, 20 nt, synthetic construct
  source 1..20: mol_type = other RNA
ctcaagtcctgtgctcctga

SEQ ID NO: 24537 - RNA, 20 nt, synthetic construct
  source 1..20: mol_type = other RNA
acaggacttgagagcacttc

SEQ ID NO: 24538 - RNA, 20 nt, synthetic construct
  source 1..20: mol_type = other RNA
caggacttgagagcacttct

SEQ ID NO: 24539 - RNA, 20 nt, synthetic construct
  source 1..20: mol_type = other RNA
gacttgagagcacttctggg

SEQ ID NO: 24540 - RNA, 20 nt, synthetic construct
  source 1..20: mol_type = other RNA
acttgagagcacttctgggt

SEQ ID NO: 24541 - RNA, 20 nt, synthetic construct
  source 1..20: mol_type = other RNA
gggtgggaacagacccagcc

SEQ ID NO: 24542 - RNA, 20 nt, synthetic construct
  source 1..20: mol_type = other RNA
ggtgggaacagacccagcct

SEQ ID NO: 24543 - RNA, 20 nt, synthetic construct
  source 1..20: mol_type = other RNA
gtgggaacagacccagcctg

SEQ ID NO: 24544 - RNA, 20 nt, synthetic construct
  source 1..20: mol_type = other RNA
gaacagacccagcctggggc

SEQ ID NO: 24545 - RNA, 20 nt, synthetic construct
  source 1..20: mol_type = other RNA
aacagacccagcctggggca

SEQ ID NO: 24546 - RNA, 20 nt, synthetic construct
  source 1..20: mol_type = other RNA
cccagcctggggcagggctc

SEQ ID NO: 24547 - RNA, 20 nt, synthetic construct
  source 1..20: mol_type = other RNA
cctgagccctgccccaggct

SEQ ID NO: 24548 - RNA, 20 nt, synthetic construct
  source 1..20: mol_type = other RNA
acctgagccctgccccaggc

SEQ ID NO: 24549 - RNA, 20 nt, synthetic construct
  source 1..20: mol_type = other RNA
agaaacctgagccctgcccc

SEQ ID NO: 24550 - RNA, 20 nt, synthetic construct
  source 1..20: mol_type = other RNA
gcagggctcaggtttctgat

SEQ ID NO: 24551 - RNA, 20 nt, synthetic construct
  source 1..20: mol_type = other RNA
caggtttctgatgggaattc

SEQ ID NO: 24552 - RNA, 20 nt, synthetic construct
  source 1..20: mol_type = other RNA
tttctgatgggaattctgga

SEQ ID NO: 24553 - RNA, 20 nt, synthetic construct
  source 1..20: mol_type = other RNA
ttctgatgggaattctggaa

SEQ ID NO: 24554 - RNA, 20 nt, synthetic construct
  source 1..20: mol_type = other RNA
ttgaagcatgttgaataaaa

SEQ ID NO: 24555 - RNA, 20 nt, synthetic construct
  source 1..20: mol_type = other RNA
attgaagcatgttgaataaa

SEQ ID NO: 24556 - RNA, 20 nt, synthetic construct
  source 1..20: mol_type = other RNA
attcaacatgcttcaatcca

SEQ ID NO: 24557 - RNA, 20 nt, synthetic construct
  source 1..20: mol_type = other RNA
ttcaacatgcttcaatccag

SEQ ID NO: 24558 - RNA, 20 nt, synthetic construct
  source 1..20: mol_type = other RNA
ggtcagacttcgggggcccc

SEQ ID NO: 24559 - RNA, 20 nt, synthetic construct
  source 1..20: mol_type = other RNA
ttgctgtggtcagacttcgg

SEQ ID NO: 24560 - RNA, 20 nt, synthetic construct
  source 1..20: mol_type = other RNA
attgctgtggtcagacttcg

SEQ ID NO: 24561 - RNA, 20 nt, synthetic construct
  source 1..20: mol_type = other RNA
cattgctgtggtcagacttc

SEQ ID NO: 24562 - RNA, 20 nt, synthetic construct
  source 1..20: mol_type = other RNA
gcattgctgtggtcagactt

SEQ ID NO: 24563 - RNA, 20 nt, synthetic construct
  source 1..20: mol_type = other RNA
catggtttggagcattgctg

SEQ ID NO: 24564 - RNA, 20 nt, synthetic construct
  source 1..20: mol_type = other RNA
tccaaaccatgtgtctttcc

SEQ ID NO: 24565 - RNA, 20 nt, synthetic construct
  source 1..20: mol_type = other RNA
gccaggaaagacacatggtt

SEQ ID NO: 24566 - RNA, 20 nt, synthetic construct
  source 1..20: mol_type = other RNA
catgtgtctttcctggctta

SEQ ID NO: 24567 - RNA, 20 nt, synthetic construct
  source 1..20: mol_type = other RNA
cttaagccaggaaagacaca

SEQ ID NO: 24568 - RNA, 20 nt, synthetic construct
  source 1..20: mol_type = other RNA
gggcgactgaaccttaagcc

SEQ ID NO: 24569 - RNA, 20 nt, synthetic construct
  source 1..20: mol_type = other RNA
ggttcagtcgccctcctcag

SEQ ID NO: 24570 - RNA, 20 nt, synthetic construct
  source 1..20: mol_type = other RNA
gttcagtcgccctcctcaga

SEQ ID NO: 24571 - RNA, 20 nt, synthetic construct
  source 1..20: mol_type = other RNA
ttcagtcgccctcctcagag

SEQ ID NO: 24572 - RNA, 20 nt, synthetic construct
  source 1..20: mol_type = other RNA
cataggctcccctctgagga

SEQ ID NO: 24573 - RNA, 20 nt, synthetic construct
  source 1..20: mol_type = other RNA
tcataggctcccctctgagg

SEQ ID NO: 24574 - RNA, 20 nt, synthetic construct
  source 1..20: mol_type = other RNA
ctttcataggctcccctctg

SEQ ID NO: 24575 - RNA, 20 nt, synthetic construct
  source 1..20: mol_type = other RNA
gagcctatgaaagagcccag

SEQ ID NO: 24576 - RNA, 20 nt, synthetic construct
  source 1..20: mol_type = other RNA
actccactgggctctttcat

SEQ ID NO: 24577 - RNA, 20 nt, synthetic construct
  source 1..20: mol_type = other RNA
aaagagcccagtggagtgtc

SEQ ID NO: 24578 - RNA, 20 nt, synthetic construct
  source 1..20: mol_type = other RNA
aagagcccagtggagtgtca

SEQ ID NO: 24579 - RNA, 20 nt, synthetic construct
  source 1..20: mol_type = other RNA
caggaccctgacactccact

SEQ ID NO: 24580 - RNA, 20 nt, synthetic construct
  source 1..20: mol_type = other RNA
tcaggaccctgacactccac

SEQ ID NO: 24581 - RNA, 20 nt, synthetic construct
  source 1..20: mol_type = other RNA
caggactaggactaggactc

SEQ ID NO: 24582 - RNA, 20 nt, synthetic construct
  source 1..20: mol_type = other RNA
gcagggacaggactaggact

SEQ ID NO: 24583 - RNA, 20 nt, synthetic construct
  source 1..20: mol_type = other RNA
caagtggcagggacaggact

SEQ ID NO: 24584 - RNA, 20 nt, synthetic construct
  source 1..20: mol_type = other RNA
cctgtccctgccacttgtga

SEQ ID NO: 24585 - RNA, 20 nt, synthetic construct
  source 1..20: mol_type = other RNA
ccctcacaagtggcagggac

SEQ ID NO: 24586 - RNA, 20 nt, synthetic construct
  source 1..20: mol_type = other RNA
ctgccacttgtgagggaact

SEQ ID NO: 24587 - RNA, 20 nt, synthetic construct
  source 1..20: mol_type = other RNA
tgccacttgtgagggaactt

SEQ ID NO: 24588 - RNA, 20 nt, synthetic construct
  source 1..20: mol_type = other RNA
aagttccctcacaagtggca

SEQ ID NO: 24589 - RNA, 20 nt, synthetic construct
  source 1..20: mol_type = other RNA
caagttccctcacaagtggc

SEQ ID NO: 24590 - RNA, 20 nt, synthetic construct
  source 1..20: mol_type = other RNA
ggcccaagttccctcacaag

SEQ ID NO: 24591 - RNA, 20 nt, synthetic construct
  source 1..20: mol_type = other RNA
acttgggcctcagtttctcc

SEQ ID NO: 24592 - RNA, 20 nt, synthetic construct
  source 1..20: mol_type = other RNA
tgggcctcagtttctccagg

SEQ ID NO: 24593 - RNA, 20 nt, synthetic construct
  source 1..20: mol_type = other RNA
gggcctcagtttctccaggt

SEQ ID NO: 24594 - RNA, 20 nt, synthetic construct
  source 1..20: mol_type = other RNA
gagcccacctggagaaactg

SEQ ID NO: 24595 - RNA, 20 nt, synthetic construct
  source 1..20: mol_type = other RNA
aagcaattgtggagcccacc

SEQ ID NO: 24596 - RNA, 20 nt, synthetic construct
  source 1..20: mol_type = other RNA
cacaattgcttctcttgatc

SEQ ID NO: 24597 - RNA, 20 nt, synthetic construct
  source 1..20: mol_type = other RNA
cagatcaagagaagcaattg

SEQ ID NO: 24598 - RNA, 20 nt, synthetic construct
  source 1..20: mol_type = other RNA
tctggactgccccagtgccc

SEQ ID NO: 24599 - RNA, 20 nt, synthetic construct
  source 1..20: mol_type = other RNA
ctcactgaacctgggcactg

SEQ ID NO: 24600 - RNA, 20 nt, synthetic construct
  source 1..20: mol_type = other RNA
actcactgaacctgggcact

SEQ ID NO: 24601 - RNA, 20 nt, synthetic construct
  source 1..20: mol_type = other RNA
cactcactgaacctgggcac

SEQ ID NO: 24602 - RNA, 20 nt, synthetic construct
  source 1..20: mol_type = other RNA
ccaggttcagtgagtgacac

SEQ ID NO: 24603 - RNA, 20 nt, synthetic construct
  source 1..20: mol_type = other RNA
ctgtgtcactcactgaacct

SEQ ID NO: 24604 - RNA, 20 nt, synthetic construct
  source 1..20: mol_type = other RNA
cctgtgtcactcactgaacc

SEQ ID NO: 24605 - RNA, 20 nt, synthetic construct
  source 1..20: mol_type = other RNA
cagtgagtgacacaggcagc

SEQ ID NO: 24606 - RNA, 20 nt, synthetic construct
  source 1..20: mol_type = other RNA
agtgagtgacacaggcagct

SEQ ID NO: 24607 - RNA, 20 nt, synthetic construct
  source 1..20: mol_type = other RNA
ggtttccacatcctctgact

SEQ ID NO: 24608 - RNA, 20 nt, synthetic construct
  source 1..20: mol_type = other RNA
gtttccacatcctctgactt

SEQ ID NO: 24609 - RNA, 20 nt, synthetic construct
  source 1..20: mol_type = other RNA
ggaacccaagtcagaggatg

SEQ ID NO: 24610 - RNA, 20 nt, synthetic construct
  source 1..20: mol_type = other RNA
gtgaagggaacccaagtcag

SEQ ID NO: 24611 - RNA, 20 nt, synthetic construct
  source 1..20: mol_type = other RNA
gggttcccttcactgcctcc

SEQ ID NO: 24612 - RNA, 20 nt, synthetic construct
  source 1..20: mol_type = other RNA
tcccttcactgcctccaggc

SEQ ID NO: 24613 - RNA, 20 nt, synthetic construct
  source 1..20: mol_type = other RNA
cccttcactgcctccaggca

SEQ ID NO: 24614 - RNA, 20 nt, synthetic construct
  source 1..20: mol_type = other RNA
ccctgcctggaggcagtgaa

SEQ ID NO: 24615 - RNA, 20 nt, synthetic construct
  source 1..20: mol_type = other RNA
gccctgcctggaggcagtga

SEQ ID NO: 24616 - RNA, 20 nt, synthetic construct
  source 1..20: mol_type = other RNA
gagggccgagccctgcctgg

SEQ ID NO: 24617 - RNA, 20 nt, synthetic construct
  source 1..20: mol_type = other RNA
gtggagggccgagccctgcc

SEQ ID NO: 24618 - RNA, 20 nt, synthetic construct
  source 1..20: mol_type = other RNA
ctcggccctccacccccaag

SEQ ID NO: 24619 - RNA, 20 nt, synthetic construct
  source 1..20: mol_type = other RNA
atgggccacttgggggtgga

SEQ ID NO: 24620 - RNA, 20 nt, synthetic construct
  source 1..20: mol_type = other RNA
aatgggccacttgggggtgg

SEQ ID NO: 24621 - RNA, 20 nt, synthetic construct
  source 1..20: mol_type = other RNA
cacaatgggccacttggggg

SEQ ID NO: 24622 - RNA, 20 nt, synthetic construct
  source 1..20: mol_type = other RNA
tcacacaatgggccacttgg

SEQ ID NO: 24623 - RNA, 20 nt, synthetic construct
  source 1..20: mol_type = other RNA
ctcacacaatgggccacttg

SEQ ID NO: 24624 - RNA, 20 nt, synthetic construct
  source 1..20: mol_type = other RNA
gctcacacaatgggccactt

SEQ ID NO: 24625 - RNA, 20 nt, synthetic construct
  source 1..20: mol_type = other RNA
agctcacacaatgggccact

SEQ ID NO: 24626 - RNA, 20 nt, synthetic construct
  source 1..20: mol_type = other RNA
ttgtgtgagctcagtttcag

SEQ ID NO: 24627 - RNA, 20 nt, synthetic construct
  source 1..20: mol_type = other RNA
tgaaactgagctcacacaat

SEQ ID NO: 24628 - RNA, 20 nt, synthetic construct
  source 1..20: mol_type = other RNA
gtgtgagctcagtttcagtg

SEQ ID NO: 24629 - RNA, 20 nt, synthetic construct
  source 1..20: mol_type = other RNA
gtttcagtggggacagaaac

SEQ ID NO: 24630 - RNA, 20 nt, synthetic construct
  source 1..20: mol_type = other RNA
tttcagtggggacagaaact

SEQ ID NO: 24631 - RNA, 20 nt, synthetic construct
  source 1..20: mol_type = other RNA
acagaaactgggttgagaaa

SEQ ID NO: 24632 - RNA, 20 nt, synthetic construct
  source 1..20: mol_type = other RNA
cagaaactgggttgagaaaa

SEQ ID NO: 24633 - RNA, 20 nt, synthetic construct
  source 1..20: mol_type = other RNA
tggcattggcttggtgggat

SEQ ID NO: 24634 - RNA, 20 nt, synthetic construct
  source 1..20: mol_type = other RNA
ttacttggcattggcttggt

SEQ ID NO: 24635 - RNA, 20 nt, synthetic construct
  source 1..20: mol_type = other RNA
tttacttggcattggcttgg

SEQ ID NO: 24636 - RNA, 20 nt, synthetic construct
  source 1..20: mol_type = other RNA
ctatttacttggcattggct

SEQ ID NO: 24637 - RNA, 20 nt, synthetic construct
  source 1..20: mol_type = other RNA
ctgcactatttacttggcat

SEQ ID NO: 24638 - RNA, 20 nt, synthetic construct
  source 1..20: mol_type = other RNA
aagatactgcactatttact

SEQ ID NO: 24639 - RNA, 20 nt, synthetic construct
  source 1..20: mol_type = other RNA
ttgccctgcccttccccatc

SEQ ID NO: 24640 - RNA, 20 nt, synthetic construct
  source 1..20: mol_type = other RNA
tgccctgcccttccccatct

SEQ ID NO: 24641 - RNA, 20 nt, synthetic construct
  source 1..20: mol_type = other RNA
gatggggaagggcagggcaa

SEQ ID NO: 24642 - RNA, 20 nt, synthetic construct
  source 1..20: mol_type = other RNA
agatggggaagggcagggca

SEQ ID NO: 24643 - RNA, 20 nt, synthetic construct
  source 1..20: mol_type = other RNA
cacccagatggggaagggca

SEQ ID NO: 24644 - RNA, 20 nt, synthetic construct
  source 1..20: mol_type = other RNA
gcacccagatggggaagggc

SEQ ID NO: 24645 - RNA, 20 nt, synthetic construct
  source 1..20: mol_type = other RNA
agcagcacccagatggggaa

SEQ ID NO: 24646 - RNA, 20 nt, synthetic construct
  source 1..20: mol_type = other RNA
cagcagcacccagatgggga

SEQ ID NO: 24647 - RNA, 20 nt, synthetic construct
  source 1..20: mol_type = other RNA
taggcagcagcacccagatg

SEQ ID NO: 24648 - RNA, 20 nt, synthetic construct
  source 1..20: mol_type = other RNA
ctaggcagcagcacccagat

SEQ ID NO: 24649 - RNA, 20 nt, synthetic construct
  source 1..20: mol_type = other RNA
tctaggcagcagcacccaga

SEQ ID NO: 24650 - RNA, 20 nt, synthetic construct
  source 1..20: mol_type = other RNA
tgctgcctagagcatataaa

SEQ ID NO: 24651 - RNA, 20 nt, synthetic construct
  source 1..20: mol_type = other RNA
aggtgccttttatatgctct

SEQ ID NO: 24652 - RNA, 20 nt, synthetic construct
  source 1..20: mol_type = other RNA
gcatataaaaggcaccttgc

SEQ ID NO: 24653 - RNA, 20 nt, synthetic construct
  source 1..20: mol_type = other RNA
catataaaaggcaccttgct

SEQ ID NO: 24654 - RNA, 20 nt, synthetic construct
  source 1..20: mol_type = other RNA
agtatgagacatgcccagca

SEQ ID NO: 24655 - RNA, 20 nt, synthetic construct
  source 1..20: mol_type = other RNA
tagcccaccagactcagaga

SEQ ID NO: 24656 - RNA, 20 nt, synthetic construct
  source 1..20: mol_type = other RNA
gttccgtctctgagtctggt

SEQ ID NO: 24657 - RNA, 20 nt, synthetic construct
  source 1..20: mol_type = other RNA
ggttccgtctctgagtctgg

SEQ ID NO: 24658 - RNA, 20 nt, synthetic construct
  source 1..20: mol_type = other RNA
ctcagagacggaaccagaga

SEQ ID NO: 24659 - RNA, 20 nt, synthetic construct
  source 1..20: mol_type = other RNA
tcagagacggaaccagagac

SEQ ID NO: 24660 - RNA, 20 nt, synthetic construct
  source 1..20: mol_type = other RNA
gggatgctctggcccgtctc

SEQ ID NO: 24661 - RNA, 20 nt, synthetic construct
  source 1..20: mol_type = other RNA
ggtggaggagggggatgctc

SEQ ID NO: 24662 - RNA, 20 nt, synthetic construct
  source 1..20: mol_type = other RNA
gagtttcatggtggaggagg

SEQ ID NO: 24663 - RNA, 20 nt, synthetic construct
  source 1..20: mol_type = other RNA
cgagtttcatggtggaggag

SEQ ID NO: 24664 - RNA, 20 nt, synthetic construct
  source 1..20: mol_type = other RNA
gcgagtttcatggtggagga

SEQ ID NO: 24665 - RNA, 20 nt, synthetic construct
  source 1..20: mol_type = other RNA
agcgagtttcatggtggagg

SEQ ID NO: 24666 - RNA, 20 nt, synthetic construct
  source 1..20: mol_type = other RNA
gacagcgagtttcatggtgg

SEQ ID NO: 24667 - RNA, 20 nt, synthetic construct
  source 1..20: mol_type = other RNA
ggtgacagcgagtttcatgg

SEQ ID NO: 24668 - RNA, 20 nt, synthetic construct
  source 1..20: mol_type = other RNA
gagggtgacagcgagtttca

SEQ ID NO: 24669 - RNA, 20 nt, synthetic construct
  source 1..20: mol_type = other RNA
actcgctgtcaccctcaccc

SEQ ID NO: 24670 - RNA, 20 nt, synthetic construct
  source 1..20: mol_type = other RNA
caccctcaccctggtcacac

SEQ ID NO: 24671 - RNA, 20 nt, synthetic construct
  source 1..20: mol_type = other RNA
agccagtgtgaccagggtga

SEQ ID NO: 24672 - RNA, 20 nt, synthetic construct
  source 1..20: mol_type = other RNA
gagccagtgtgaccagggtg

SEQ ID NO: 24673 - RNA, 20 nt, synthetic construct
  source 1..20: mol_type = other RNA
gcagagagccagtgtgacca

SEQ ID NO: 24674 - RNA, 20 nt, synthetic construct
  source 1..20: mol_type = other RNA
agcagagagccagtgtgacc

SEQ ID NO: 24675 - RNA, 20 nt, synthetic construct
  source 1..20: mol_type = other RNA
ctggctctctgctgcagctc

SEQ ID NO: 24676 - RNA, 20 nt, synthetic construct
  source 1..20: mol_type = other RNA
aagggtctctgagcactcac

SEQ ID NO: 24677 - RNA, 20 nt, synthetic construct
  source 1..20: mol_type = other RNA
agagacccttccctccctcc

SEQ ID NO: 24678 - RNA, 20 nt, synthetic construct
  source 1..20: mol_type = other RNA
cttccctccctcctggactt

SEQ ID NO: 24679 - RNA, 20 nt, synthetic construct
  source 1..20: mol_type = other RNA
taagtccaggagggagggaa

SEQ ID NO: 24680 - RNA, 20 nt, synthetic construct
  source 1..20: mol_type = other RNA
ctaagtccaggagggaggga

SEQ ID NO: 24681 - RNA, 20 nt, synthetic construct
  source 1..20: mol_type = other RNA
gttcctaagtccaggaggga

SEQ ID NO: 24682 - RNA, 20 nt, synthetic construct
  source 1..20: mol_type = other RNA
agttcctaagtccaggaggg

SEQ ID NO: 24683 - RNA, 20 nt, synthetic construct
  source 1..20: mol_type = other RNA
tcctggacttaggaactctc

SEQ ID NO: 24684 - RNA, 20 nt, synthetic construct
  source 1..20: mol_type = other RNA
gagagttcctaagtccagga

SEQ ID NO: 24685 - RNA, 20 nt, synthetic construct
  source 1..20: mol_type = other RNA
tgagagttcctaagtccagg

SEQ ID NO: 24686 - RNA, 20 nt, synthetic construct
  source 1..20: mol_type = other RNA
tcctgagagttcctaagtcc

SEQ ID NO: 24687 - RNA, 20 nt, synthetic construct
  source 1..20: mol_type = other RNA
ccccagttctgctcagaaga

SEQ ID NO: 24688 - RNA, 20 nt, synthetic construct
  source 1..20: mol_type = other RNA
ttcttctgagcagaactggg

SEQ ID NO: 24689 - RNA, 20 nt, synthetic construct
  source 1..20: mol_type = other RNA
cttcttctgagcagaactgg

SEQ ID NO: 24690 - RNA, 20 nt, synthetic construct
  source 1..20: mol_type = other RNA
ccttcttctgagcagaactg

SEQ ID NO: 24691 - RNA, 20 nt, synthetic construct
  source 1..20: mol_type = other RNA
tccttcttctgagcagaact

SEQ ID NO: 24692 - RNA, 20 nt, synthetic construct
  source 1..20: mol_type = other RNA
ctccttcttctgagcagaac

SEQ ID NO: 24693 - RNA, 20 nt, synthetic construct
  source 1..20: mol_type = other RNA
tgagctgcccattcctgctc

SEQ ID NO: 24694 - RNA, 20 nt, synthetic construct
  source 1..20: mol_type = other RNA
cattcctgctctggagctgc

SEQ ID NO: 24695 - RNA, 20 nt, synthetic construct
  source 1..20: mol_type = other RNA
attcctgctctggagctgct

SEQ ID NO: 24696 - RNA, 20 nt, synthetic construct
  source 1..20: mol_type = other RNA
agcagctccagagcaggaat

SEQ ID NO: 24697 - RNA, 20 nt, synthetic construct
  source 1..20: mol_type = other RNA
cctgctctggagctgctggg

SEQ ID NO: 24698 - RNA, 20 nt, synthetic construct
  source 1..20: mol_type = other RNA
cctcccagcagctccagagc

SEQ ID NO: 24699 - RNA, 20 nt, synthetic construct
  source 1..20: mol_type = other RNA
ctggagctgctgggaggacc

SEQ ID NO: 24700 - RNA, 20 nt, synthetic construct
  source 1..20: mol_type = other RNA
tggagctgctgggaggacct

SEQ ID NO: 24701 - RNA, 20 nt, synthetic construct
  source 1..20: mol_type = other RNA
aggctgctatctctcgctga

SEQ ID NO: 24702 - RNA, 20 nt, synthetic construct
  source 1..20: mol_type = other RNA
ggctgctatctctcgctgat

SEQ ID NO: 24703 - RNA, 20 nt, synthetic construct
  source 1..20: mol_type = other RNA
ctatctctcgctgatgggcc

SEQ ID NO: 24704 - RNA, 20 nt, synthetic construct
  source 1..20: mol_type = other RNA
tgggcctggctgtttgcatc

SEQ ID NO: 24705 - RNA, 20 nt, synthetic construct
  source 1..20: mol_type = other RNA
gggcctggctgtttgcatct

SEQ ID NO: 24706 - RNA, 20 nt, synthetic construct
  source 1..20: mol_type = other RNA
ctgcccagatgcaaacagcc

SEQ ID NO: 24707 - RNA, 20 nt, synthetic construct
  source 1..20: mol_type = other RNA
atctgggcagacccagccag

SEQ ID NO: 24708 - RNA, 20 nt, synthetic construct
  source 1..20: mol_type = other RNA
tctgggcagacccagccaga

SEQ ID NO: 24709 - RNA, 20 nt, synthetic construct
  source 1..20: mol_type = other RNA
agccagagggctagccagct

SEQ ID NO: 24710 - RNA, 20 nt, synthetic construct
  source 1..20: mol_type = other RNA
agctggctagccctctggct

SEQ ID NO: 24711 - RNA, 20 nt, synthetic construct
  source 1..20: mol_type = other RNA
aagctggctagccctctggc

SEQ ID NO: 24712 - RNA, 20 nt, synthetic construct
  source 1..20: mol_type = other RNA
gagggctagccagcttggaa

SEQ ID NO: 24713 - RNA, 20 nt, synthetic construct
  source 1..20: mol_type = other RNA
agggctagccagcttggaaa

SEQ ID NO: 24714 - RNA, 20 nt, synthetic construct
  source 1..20: mol_type = other RNA
gggctagccagcttggaaag

SEQ ID NO: 24715 - RNA, 20 nt, synthetic construct
  source 1..20: mol_type = other RNA
agccagcttggaaaggggcc

SEQ ID NO: 24716 - RNA, 20 nt, synthetic construct
  source 1..20: mol_type = other RNA
ctccaggcccctttccaagc

SEQ ID NO: 24717 - RNA, 20 nt, synthetic construct
  source 1..20: mol_type = other RNA
gagagaaggcacatgtctcc

SEQ ID NO: 24718 - RNA, 20 nt, synthetic construct
  source 1..20: mol_type = other RNA
gctgcaacacagaggagaga

SEQ ID NO: 24719 - RNA, 20 nt, synthetic construct
  source 1..20: mol_type = other RNA
ctgcagaagctgcaacacag

SEQ ID NO: 24720 - RNA, 20 nt, synthetic construct
  source 1..20: mol_type = other RNA
cgatgacacgctgaaagctc

SEQ ID NO: 24721 - RNA, 20 nt, synthetic construct
  source 1..20: mol_type = other RNA
tcgatgacacgctgaaagct

SEQ ID NO: 24722 - RNA, 20 nt, synthetic construct
  source 1..20: mol_type = other RNA
tgtcatcgaaaccctcctca

SEQ ID NO: 24723 - RNA, 20 nt, synthetic construct
  source 1..20: mol_type = other RNA
ggagggtgtgtccatgagga

SEQ ID NO: 24724 - RNA, 20 nt, synthetic construct
  source 1..20: mol_type = other RNA
tggagggtgtgtccatgagg

SEQ ID NO: 24725 - RNA, 20 nt, synthetic construct
  source 1..20: mol_type = other RNA
aactggagggtgtgtccatg

SEQ ID NO: 24726 - RNA, 20 nt, synthetic construct
  source 1..20: mol_type = other RNA
ggacacaccctccagttatg

SEQ ID NO: 24727 - RNA, 20 nt, synthetic construct
  source 1..20: mol_type = other RNA
ctccagttatgaggctgcca

SEQ ID NO: 24728 - RNA, 20 nt, synthetic construct
  source 1..20: mol_type = other RNA
atggcagcctcataactgga

SEQ ID NO: 24729 - RNA, 20 nt, synthetic construct
  source 1..20: mol_type = other RNA
catggcagcctcataactgg

SEQ ID NO: 24730 - RNA, 20 nt, synthetic construct
  source 1..20: mol_type = other RNA
ttccatggcagcctcataac

SEQ ID NO: 24731 - RNA, 20 nt, synthetic construct
  source 1..20: mol_type = other RNA
atcagggctgaaaagttcca

SEQ ID NO: 24732 - RNA, 20 nt, synthetic construct
  source 1..20: mol_type = other RNA
tcagccctgatcaagacatg

SEQ ID NO: 24733 - RNA, 20 nt, synthetic construct
  source 1..20: mol_type = other RNA
cagccctgatcaagacatga

SEQ ID NO: 24734 - RNA, 20 nt, synthetic construct
  source 1..20: mol_type = other RNA
ccctgatcaagacatgaggg

SEQ ID NO: 24735 - RNA, 20 nt, synthetic construct
  source 1..20: mol_type = other RNA
gatcaagacatgagggaggc

SEQ ID NO: 24736 - RNA, 20 nt, synthetic construct
  source 1..20: mol_type = other RNA
cctccctcatgtcttgatca

SEQ ID NO: 24737 - RNA, 20 nt, synthetic construct
  source 1..20: mol_type = other RNA
gcctccctcatgtcttgatc

SEQ ID NO: 24738 - RNA, 20 nt, synthetic construct
  source 1..20: mol_type = other RNA
aggggctcagctgaagaagc

SEQ ID NO: 24739 - RNA, 20 nt, synthetic construct
  source 1..20: mol_type = other RNA
ggctcagctgaagaagctgg

SEQ ID NO: 24740 - RNA, 20 nt, synthetic construct
  source 1..20: mol_type = other RNA
ttctctgggcttttggggga

SEQ ID NO: 24741 - RNA, 20 nt, synthetic construct
  source 1..20: mol_type = other RNA
tttctctgggcttttggggg

SEQ ID NO: 24742 - RNA, 20 nt, synthetic construct
  source 1..20: mol_type = other RNA
tgctttctctgggcttttgg

SEQ ID NO: 24743 - RNA, 20 nt, synthetic construct
  source 1..20: mol_type = other RNA
atgctttctctgggcttttg

SEQ ID NO: 24744 - RNA, 20 nt, synthetic construct
  source 1..20: mol_type = other RNA
gatgctttctctgggctttt

SEQ ID NO: 24745 - RNA, 20 nt, synthetic construct
  source 1..20: mol_type = other RNA
tgatgctttctctgggcttt

SEQ ID NO: 24746 - RNA, 20 nt, synthetic construct
  source 1..20: mol_type = other RNA
agaaagcatcattaagctca

SEQ ID NO: 24747 - RNA, 20 nt, synthetic construct
  source 1..20: mol_type = other RNA
gagcttaatgatgctttctc

SEQ ID NO: 24748 - RNA, 20 nt, synthetic construct
  source 1..20: mol_type = other RNA
cagcacctttcacgtcacac

SEQ ID NO: 24749 - RNA, 20 nt, synthetic construct
  source 1..20: mol_type = other RNA
cagtgtgacgtgaaaggtgc

SEQ ID NO: 24750 - RNA, 20 nt, synthetic construct
  source 1..20: mol_type = other RNA
cacgtcacactggttagaag

SEQ ID NO: 24751 - RNA, 20 nt, synthetic construct
  source 1..20: mol_type = other RNA
ttagaagtggcttccccaag

SEQ ID NO: 24752 - RNA, 20 nt, synthetic construct
  source 1..20: mol_type = other RNA
tagaagtggcttccccaagt

SEQ ID NO: 24753 - RNA, 20 nt, synthetic construct
  source 1..20: mol_type = other RNA
agaagtggcttccccaagtg

SEQ ID NO: 24754 - RNA, 20 nt, synthetic construct
  source 1..20: mol_type = other RNA
gcttccccaagtggggctgc

SEQ ID NO: 24755 - RNA, 20 nt, synthetic construct
  source 1..20: mol_type = other RNA
caatcctgcagccccacttg

SEQ ID NO: 24756 - RNA, 20 nt, synthetic construct
  source 1..20: mol_type = other RNA
gcaatcctgcagccccactt

SEQ ID NO: 24757 - RNA, 20 nt, synthetic construct
  source 1..20: mol_type = other RNA
ggcaatcctgcagccccact

SEQ ID NO: 24758 - RNA, 20 nt, synthetic construct
  source 1..20: mol_type = other RNA
agaaacaggtctgaaaactg

SEQ ID NO: 24759 - RNA, 20 nt, synthetic construct
  source 1..20: mol_type = other RNA
tagaaacaggtctgaaaact

SEQ ID NO: 24760 - RNA, 20 nt, synthetic construct
  source 1..20: mol_type = other RNA
ttagaaacaggtctgaaaac

SEQ ID NO: 24761 - RNA, 20 nt, synthetic construct
  source 1..20: mol_type = other RNA
gacctgtttctaatccagag

SEQ ID NO: 24762 - RNA, 20 nt, synthetic construct
  source 1..20: mol_type = other RNA
ctcctctctggattagaaac

SEQ ID NO: 24763 - RNA, 20 nt, synthetic construct
  source 1..20: mol_type = other RNA
ggcactgtgactctcctctc

SEQ ID NO: 24764 - RNA, 20 nt, synthetic construct
  source 1..20: mol_type = other RNA
gtcacagtgccactgtcccc

SEQ ID NO: 24765 - RNA, 20 nt, synthetic construct
  source 1..20: mol_type = other RNA
ctagagttgactgcacctct

SEQ ID NO: 24766 - RNA, 20 nt, synthetic construct
  source 1..20: mol_type = other RNA
gaggtgcagtcaactctagg

SEQ ID NO: 24767 - RNA, 20 nt, synthetic construct
  source 1..20: mol_type = other RNA
cgagaggtgcagtcaactct

SEQ ID NO: 24768 - RNA, 20 nt, synthetic construct
  source 1..20: mol_type = other RNA
aaacttcaacattaaccgag

SEQ ID NO: 24769 - RNA, 20 nt, synthetic construct
  source 1..20: mol_type = other RNA
ggttaatgttgaagtttctg

SEQ ID NO: 24770 - RNA, 20 nt, synthetic construct
  source 1..20: mol_type = other RNA
agtgaatgaattgcatagtt

SEQ ID NO: 24771 - RNA, 20 nt, synthetic construct
  source 1..20: mol_type = other RNA
caattcattcactgttgtat

SEQ ID NO: 24772 - RNA, 20 nt, synthetic construct
  source 1..20: mol_type = other RNA
aattcattcactgttgtatt

SEQ ID NO: 24773 - RNA, 20 nt, synthetic construct
  source 1..20: mol_type = other RNA
tttctttgtctatttgtttt

SEQ ID NO: 24774 - RNA, 20 nt, synthetic construct
  source 1..20: mol_type = other RNA
ctaattacacagtgagcttt

SEQ ID NO: 24775 - RNA, 20 nt, synthetic construct
  source 1..20: mol_type = other RNA
gctaattacacagtgagctt

SEQ ID NO: 24776 - RNA, 20 nt, synthetic construct
  source 1..20: mol_type = other RNA
ggcagaggctggagcagttg

SEQ ID NO: 24777 - RNA, 20 nt, synthetic construct
  source 1..20: mol_type = other RNA
cggcagaggctggagcagtt

SEQ ID NO: 24778 - RNA, 20 nt, synthetic construct
  source 1..20: mol_type = other RNA
gcggcagaggctggagcagt

SEQ ID NO: 24779 - RNA, 20 nt, synthetic construct
  source 1..20: mol_type = other RNA
agcatggcagcggcagaggc

SEQ ID NO: 24780 - RNA, 20 nt, synthetic construct
  source 1..20: mol_type = other RNA
tcaaagcatggcagcggcag

SEQ ID NO: 24781 - RNA, 20 nt, synthetic construct
  source 1..20: mol_type = other RNA
gtggactcaaagcatggcag

SEQ ID NO: 24782 - RNA, 20 nt, synthetic construct
  source 1..20: mol_type = other RNA
gtgggcgtggactcaaagca

SEQ ID NO: 24783 - RNA, 20 nt, synthetic construct
  source 1..20: mol_type = other RNA
gagagcaaggctggtgggcg

SEQ ID NO: 24784 - RNA, 20 nt, synthetic construct
  source 1..20: mol_type = other RNA
ttgaagagagcaaggctggt

SEQ ID NO: 24785 - RNA, 20 nt, synthetic construct
  source 1..20: mol_type = other RNA
attgaagagagcaaggctgg

SEQ ID NO: 24786 - RNA, 20 nt, synthetic construct
  source 1..20: mol_type = other RNA
tttattgaagagagcaaggc

SEQ ID NO: 24787 - RNA, 20 nt, synthetic construct
  source 1..20: mol_type = other RNA
gtggtttattgaagagagca

SEQ ID NO: 24788 - RNA, 20 nt, synthetic construct
  source 1..20: mol_type = other RNA
gcacaaaagtgagatgcttg

SEQ ID NO: 24789 - DNA, 28 bp, synthetic construct
  source 1..28: mol_type = other DNA
ttcgggtgaattttgagcgaggtgaagg

SEQ ID NO: 24790 - DNA, 28 bp, synthetic construct
  source 1..28: mol_type = other DNA
cgcattttcgggtgaattttgagcgagg

SEQ ID NO: 24791 - DNA, 28 bp, synthetic construct
  source 1..28: mol_type = other DNA
ttcacccgaaaatgcgctgagactttgg

SEQ ID NO: 24792 - DNA, 28 bp, synthetic construct
  source 1..28: mol_type = other DNA
catgccaaagtctcagcgcattttcggg

SEQ ID NO: 24793 - DNA, 28 bp, synthetic construct
  source 1..28: mol_type = other DNA
ccgaaaatgcgctgagactttggcatgg

SEQ ID NO: 24794 - DNA, 28 bp, synthetic construct
  source 1..28: mol_type = other DNA
cgaaaatgcgctgagactttggcatggg

SEQ ID NO: 24795 - DNA, 28 bp, synthetic construct
  source 1..28: mol_type = other DNA
gaaaatgcgctgagactttggcatgggg

SEQ ID NO: 24796 - DNA, 28 bp, synthetic construct
  source 1..28: mol_type = other DNA
tcataagcgcttctgtaacgtcagtggg

SEQ ID NO: 24797 - DNA, 28 bp, synthetic construct
  source 1..28: mol_type = other DNA
ttcataagcgcttctgtaacgtcagtgg

SEQ ID NO: 24798 - DNA, 28 bp, synthetic construct
  source 1..28: mol_type = other DNA
cgcttatgaatttaaaaactgctccagg

SEQ ID NO: 24799 - DNA, 28 bp, synthetic construct
  source 1..28: mol_type = other DNA
ttatgaatttaaaaactgctccaggcgg

SEQ ID NO: 24800 - DNA, 28 bp, synthetic construct
  source 1..28: mol_type = other DNA
gaatttaaaaactgctccaggcggccgg

SEQ ID NO: 24801 - DNA, 28 bp, synthetic construct
  source 1..28: mol_type = other DNA
ttaaaaactgctccaggcggccggacgg

SEQ ID NO: 24802 - DNA, 28 bp, synthetic construct
  source 1..28: mol_type = other DNA
aaaactgctccaggcggccggacggcgg

SEQ ID NO: 24803 - DNA, 28 bp, synthetic construct
  source 1..28: mol_type = other DNA
aaactgctccaggcggccggacggcggg

SEQ ID NO: 24804 - DNA, 28 bp, synthetic construct
  source 1..28: mol_type = other DNA
ggcgttgtcccgccgtccggccgcctgg

SEQ ID NO: 24805 - DNA, 28 bp, synthetic construct
  source 1..28: mol_type = other DNA
agtgaggaggcgttgtcccgccgtccgg

SEQ ID NO: 24806 - DNA, 28 bp, synthetic construct
  source 1..28: mol_type = other DNA
caacgcctcctcacttgctcctctacgg

SEQ ID NO: 24807 - DNA, 28 bp, synthetic construct
  source 1..28: mol_type = other DNA
ccttgccgtagaggagcaagtgaggagg

SEQ ID NO: 24808 - DNA, 28 bp, synthetic construct
  source 1..28: mol_type = other DNA
gggccttgccgtagaggagcaagtgagg

SEQ ID NO: 24809 - DNA, 28 bp, synthetic construct
  source 1..28: mol_type = other DNA
ggagaaggaaggggccttgccgtagagg

SEQ ID NO: 24810 - DNA, 28 bp, synthetic construct
  source 1..28: mol_type = other DNA
ggcaaggccccttccttctccctgccgg

SEQ ID NO: 24811 - DNA, 28 bp, synthetic construct
  source 1..28: mol_type = other DNA
gccccttccttctccctgccggctgcgg

SEQ ID NO: 24812 - DNA, 28 bp, synthetic construct
  source 1..28: mol_type = other DNA
accgcagccggcagggagaaggaagggg

SEQ ID NO: 24813 - DNA, 28 bp, synthetic construct
  source 1..28: mol_type = other DNA
caccgcagccggcagggagaaggaaggg

SEQ ID NO: 24814 - DNA, 28 bp, synthetic construct
  source 1..28: mol_type = other DNA
ccttccttctccctgccggctgcggtgg

SEQ ID NO: 24815 - DNA, 28 bp, synthetic construct
  source 1..28: mol_type = other DNA
cacaccaccgcagccggcagggagaagg

SEQ ID NO: 24816 - DNA, 28 bp, synthetic construct
  source 1..28: mol_type = other DNA
ctccctgccggctgcggtggtgtgtagg

SEQ ID NO: 24817 - DNA, 28 bp, synthetic construct
  source 1..28: mol_type = other DNA
tccctgccggctgcggtggtgtgtaggg

SEQ ID NO: 24818 - DNA, 28 bp, synthetic construct
  source 1..28: mol_type = other DNA
accctacacaccaccgcagccggcaggg

SEQ ID NO: 24819 - DNA, 28 bp, synthetic construct
  source 1..28: mol_type = other DNA
caccctacacaccaccgcagccggcagg

SEQ ID NO: 24820 - DNA, 28 bp, synthetic construct
  source 1..28: mol_type = other DNA
ctgccggctgcggtggtgtgtagggtgg

SEQ ID NO: 24821 - DNA, 28 bp, synthetic construct
  source 1..28: mol_type = other DNA
ggaccaccctacacaccaccgcagccgg

SEQ ID NO: 24822 - DNA, 28 bp, synthetic construct
  source 1..28: mol_type = other DNA
agatggattaaggaaactctgtaaaggg

SEQ ID NO: 24823 - DNA, 28 bp, synthetic construct
  source 1..28: mol_type = other DNA
tagatggattaaggaaactctgtaaagg

SEQ ID NO: 24824 - DNA, 28 bp, synthetic construct
  source 1..28: mol_type = other DNA
aggtgaggtcaggctagatggattaagg

SEQ ID NO: 24825 - DNA, 28 bp, synthetic construct
  source 1..28: mol_type = other DNA
aatccatctagcctgacctcacctgcgg

SEQ ID NO: 24826 - DNA, 28 bp, synthetic construct
  source 1..28: mol_type = other DNA
atccatctagcctgacctcacctgcggg

SEQ ID NO: 24827 - DNA, 28 bp, synthetic construct
  source 1..28: mol_type = other DNA
atcccgcaggtgaggtcaggctagatgg

SEQ ID NO: 24828 - DNA, 28 bp, synthetic construct
  source 1..28: mol_type = other DNA
aatggaacatcccgcaggtgaggtcagg

SEQ ID NO: 24829 - DNA, 28 bp, synthetic construct
  source 1..28: mol_type = other DNA
cgggaaatggaacatcccgcaggtgagg

SEQ ID NO: 24830 - DNA, 28 bp, synthetic construct
  source 1..28: mol_type = other DNA
tggatcgggaaatggaacatcccgcagg

SEQ ID NO: 24831 - DNA, 28 bp, synthetic construct
  source 1..28: mol_type = other DNA
ggggtgtgggaggtggatcgggaaatgg

SEQ ID NO: 24832 - DNA, 28 bp, synthetic construct
  source 1..28: mol_type = other DNA
gcagcgggggtgtgggaggtggatcggg

SEQ ID NO: 24833 - DNA, 28 bp, synthetic construct
  source 1..28: mol_type = other DNA
tgcagcgggggtgtgggaggtggatcgg

SEQ ID NO: 24834 - DNA, 28 bp, synthetic construct
  source 1..28: mol_type = other DNA
acaactgcagcgggggtgtgggaggtgg

SEQ ID NO: 24835 - DNA, 28 bp, synthetic construct
  source 1..28: mol_type = other DNA
tagacaactgcagcgggggtgtgggagg

SEQ ID NO: 24836 - DNA, 28 bp, synthetic construct
  source 1..28: mol_type = other DNA
ttctagacaactgcagcgggggtgtggg

SEQ ID NO: 24837 - DNA, 28 bp, synthetic construct
  source 1..28: mol_type = other DNA
cttctagacaactgcagcgggggtgtgg

SEQ ID NO: 24838 - DNA, 28 bp, synthetic construct
  source 1..28: mol_type = other DNA
acccccgctgcagttgtctagaagctgg

SEQ ID NO: 24839 - DNA, 28 bp, synthetic construct
  source 1..28: mol_type = other DNA
cccagcttctagacaactgcagcggggg

SEQ ID NO: 24840 - DNA, 28 bp, synthetic construct
  source 1..28: mol_type = other DNA
ccccgctgcagttgtctagaagctgggg

SEQ ID NO: 24841 - DNA, 28 bp, synthetic construct
  source 1..28: mol_type = other DNA
gccccagcttctagacaactgcagcggg

SEQ ID NO: 24842 - DNA, 28 bp, synthetic construct
  source 1..28: mol_type = other DNA
agccccagcttctagacaactgcagcgg

SEQ ID NO: 24843 - DNA, 28 bp, synthetic construct
  source 1..28: mol_type = other DNA
gctgcagttgtctagaagctggggctgg

SEQ ID NO: 24844 - DNA, 28 bp, synthetic construct
  source 1..28: mol_type = other DNA
ctgcagttgtctagaagctggggctggg

SEQ ID NO: 24845 - DNA, 28 bp, synthetic construct
  source 1..28: mol_type = other DNA
tgcagttgtctagaagctggggctgggg

SEQ ID NO: 24846 - DNA, 28 bp, synthetic construct
  source 1..28: mol_type = other DNA
tctagaagctggggctggggaactgagg

SEQ ID NO: 24847 - DNA, 28 bp, synthetic construct
  source 1..28: mol_type = other DNA
aagctggggctggggaactgaggcgcgg

SEQ ID NO: 24848 - DNA, 28 bp, synthetic construct
  source 1..28: mol_type = other DNA
agctggggctggggaactgaggcgcggg

SEQ ID NO: 24849 - DNA, 28 bp, synthetic construct
  source 1..28: mol_type = other DNA
tggggctggggaactgaggcgcgggagg

SEQ ID NO: 24850 - DNA, 28 bp, synthetic construct
  source 1..28: mol_type = other DNA
gaactgaggcgcgggaggagcagacagg

SEQ ID NO: 24851 - DNA, 28 bp, synthetic construct
  source 1..28: mol_type = other DNA
ctgaggcgcgggaggagcagacaggagg

SEQ ID NO: 24852 - DNA, 28 bp, synthetic construct
  source 1..28: mol_type = other DNA
tgaggcgcgggaggagcagacaggaggg

SEQ ID NO: 24853 - DNA, 28 bp, synthetic construct
  source 1..28: mol_type = other DNA
gcgcgggaggagcagacaggagggccgg

SEQ ID NO: 24854 - DNA, 28 bp, synthetic construct
  source 1..28: mol_type = other DNA
cgcgggaggagcagacaggagggccggg

SEQ ID NO: 24855 - DNA, 28 bp, synthetic construct
  source 1..28: mol_type = other DNA
gcgggaggagcagacaggagggccgggg

SEQ ID NO: 24856 - DNA, 28 bp, synthetic construct
  source 1..28: mol_type = other DNA
gaggagcagacaggagggccggggttgg

SEQ ID NO: 24857 - DNA, 28 bp, synthetic construct
  source 1..28: mol_type = other DNA
aggagcagacaggagggccggggttggg

SEQ ID NO: 24858 - DNA, 28 bp, synthetic construct
  source 1..28: mol_type = other DNA
ggagcagacaggagggccggggttgggg

SEQ ID NO: 24859 - DNA, 28 bp, synthetic construct
  source 1..28: mol_type = other DNA
caacgcgtggctggcgccccaaccccgg

SEQ ID NO: 24860 - DNA, 28 bp, synthetic construct
  source 1..28: mol_type = other DNA
cggggttggggcgccagccacgcgttgg

SEQ ID NO: 24861 - DNA, 28 bp, synthetic construct
  source 1..28: mol_type = other DNA
ggggttggggcgccagccacgcgttggg

SEQ ID NO: 24862 - DNA, 28 bp, synthetic construct
  source 1..28: mol_type = other DNA
cgggtctgctctcccaacgcgtggctgg

SEQ ID NO: 24863 - DNA, 28 bp, synthetic construct
  source 1..28: mol_type = other DNA
cagccacgcgttgggagagcagacccgg

SEQ ID NO: 24864 - DNA, 28 bp, synthetic construct
  source 1..28: mol_type = other DNA
agccacgcgttgggagagcagacccggg

SEQ ID NO: 24865 - DNA, 28 bp, synthetic construct
  source 1..28: mol_type = other DNA
cacccgggtctgctctcccaacgcgtgg

SEQ ID NO: 24866 - DNA, 28 bp, synthetic construct
  source 1..28: mol_type = other DNA
agagcagacccgggtgcagactcagagg

SEQ ID NO: 24867 - DNA, 28 bp, synthetic construct
  source 1..28: mol_type = other DNA
agacccgggtgcagactcagaggactgg

SEQ ID NO: 24868 - DNA, 28 bp, synthetic construct
  source 1..28: mol_type = other DNA
tctccagtcctctgagtctgcacccggg

SEQ ID NO: 24869 - DNA, 28 bp, synthetic construct
  source 1..28: mol_type = other DNA
ctctccagtcctctgagtctgcacccgg

SEQ ID NO: 24870 - DNA, 28 bp, synthetic construct
  source 1..28: mol_type = other DNA
cgggtgcagactcagaggactggagagg

SEQ ID NO: 24871 - DNA, 28 bp, synthetic construct
  source 1..28: mol_type = other DNA
gtgcagactcagaggactggagaggcgg

SEQ ID NO: 24872 - DNA, 28 bp, synthetic construct
  source 1..28: mol_type = other DNA
gactcagaggactggagaggcggcatgg

SEQ ID NO: 24873 - DNA, 28 bp, synthetic construct
  source 1..28: mol_type = other DNA
aggactggagaggcggcatggagtttgg

SEQ ID NO: 24874 - DNA, 28 bp, synthetic construct
  source 1..28: mol_type = other DNA
agaggcggcatggagtttggtctcctgg

SEQ ID NO: 24875 - DNA, 28 bp, synthetic construct
  source 1..28: mol_type = other DNA
gaggcggcatggagtttggtctcctggg

SEQ ID NO: 24876 - DNA, 28 bp, synthetic construct
  source 1..28: mol_type = other DNA
gcggcatggagtttggtctcctgggagg

SEQ ID NO: 24877 - DNA, 28 bp, synthetic construct
  source 1..28: mol_type = other DNA
gtttggtctcctgggaggtagagtgagg

SEQ ID NO: 24878 - DNA, 28 bp, synthetic construct
  source 1..28: mol_type = other DNA
tcctgggaggtagagtgaggtgctgcgg

SEQ ID NO: 24879 - DNA, 28 bp, synthetic construct
  source 1..28: mol_type = other DNA
tccgcagcacctcactctacctcccagg

SEQ ID NO: 24880 - DNA, 28 bp, synthetic construct
  source 1..28: mol_type = other DNA
ggtagagtgaggtgctgcggactccagg

SEQ ID NO: 24881 - DNA, 28 bp, synthetic construct
  source 1..28: mol_type = other DNA
gtagagtgaggtgctgcggactccaggg

SEQ ID NO: 24882 - DNA, 28 bp, synthetic construct
  source 1..28: mol_type = other DNA
gagtgaggtgctgcggactccagggagg

SEQ ID NO: 24883 - DNA, 28 bp, synthetic construct
  source 1..28: mol_type = other DNA
aggtgctgcggactccagggaggaaagg

SEQ ID NO: 24884 - DNA, 28 bp, synthetic construct
  source 1..28: mol_type = other DNA
ggtgctgcggactccagggaggaaaggg

SEQ ID NO: 24885 - DNA, 28 bp, synthetic construct
  source 1..28: mol_type = other DNA
ctgcggactccagggaggaaagggatgg

SEQ ID NO: 24886 - DNA, 28 bp, synthetic construct
  source 1..28: mol_type = other DNA
tgcggactccagggaggaaagggatggg

SEQ ID NO: 24887 - DNA, 28 bp, synthetic construct
  source 1..28: mol_type = other DNA
ggactccagggaggaaagggatgggtgg

SEQ ID NO: 24888 - DNA, 28 bp, synthetic construct
  source 1..28: mol_type = other DNA
gactccagggaggaaagggatgggtggg

SEQ ID NO: 24889 - DNA, 28 bp, synthetic construct
  source 1..28: mol_type = other DNA
actccagggaggaaagggatgggtgggg

SEQ ID NO: 24890 - DNA, 28 bp, synthetic construct
  source 1..28: mol_type = other DNA
ccagggaggaaagggatgggtggggagg

SEQ ID NO: 24891 - DNA, 28 bp, synthetic construct
  source 1..28: mol_type = other DNA
gggaggaaagggatgggtggggaggcgg

SEQ ID NO: 24892 - DNA, 28 bp, synthetic construct
  source 1..28: mol_type = other DNA
ggaggaaagggatgggtggggaggcggg

SEQ ID NO: 24893 - DNA, 28 bp, synthetic construct
  source 1..28: mol_type = other DNA
ggaaagggatgggtggggaggcgggagg

SEQ ID NO: 24894 - DNA, 28 bp, synthetic construct
  source 1..28: mol_type = other DNA
gaaagggatgggtggggaggcgggaggg

SEQ ID NO: 24895 - DNA, 28 bp, synthetic construct
  source 1..28: mol_type = other DNA
aaagggatgggtggggaggcgggagggg

SEQ ID NO: 24896 - DNA, 28 bp, synthetic construct
  source 1..28: mol_type = other DNA
gggatgggtggggaggcgggaggggagg

SEQ ID NO: 24897 - DNA, 28 bp, synthetic construct
  source 1..28: mol_type = other DNA
atgggtggggaggcgggaggggaggagg

SEQ ID NO: 24898 - DNA, 28 bp, synthetic construct
  source 1..28: mol_type = other DNA
tgggtggggaggcgggaggggaggaggg

SEQ ID NO: 24899 - DNA, 28 bp, synthetic construct
  source 1..28: mol_type = other DNA
tggggaggcgggaggggaggagggacgg

SEQ ID NO: 24900 - DNA, 28 bp, synthetic construct
  source 1..28: mol_type = other DNA
ggggaggcgggaggggaggagggacggg

SEQ ID NO: 24901 - DNA, 28 bp, synthetic construct
  source 1..28: mol_type = other DNA
gggaggcgggaggggaggagggacgggg

SEQ ID NO: 24902 - DNA, 28 bp, synthetic construct
  source 1..28: mol_type = other DNA
cggggtattttgcgctcccgcaccgcgg

SEQ ID NO: 24903 - DNA, 28 bp, synthetic construct
  source 1..28: mol_type = other DNA
aacagctgagttcgggccgcggtgcggg

SEQ ID NO: 24904 - DNA, 28 bp, synthetic construct
  source 1..28: mol_type = other DNA
gaacagctgagttcgggccgcggtgcgg

SEQ ID NO: 24905 - DNA, 28 bp, synthetic construct
  source 1..28: mol_type = other DNA
aggcagaacagctgagttcgggccgcgg

SEQ ID NO: 24906 - DNA, 28 bp, synthetic construct
  source 1..28: mol_type = other DNA
cagtgaaggcagaacagctgagttcggg

SEQ ID NO: 24907 - DNA, 28 bp, synthetic construct
  source 1..28: mol_type = other DNA
ccgaactcagctgttctgccttcactgg

SEQ ID NO: 24908 - DNA, 28 bp, synthetic construct
  source 1..28: mol_type = other DNA
tgccttcactggcctcagccagtcgagg

SEQ ID NO: 24909 - DNA, 28 bp, synthetic construct
  source 1..28: mol_type = other DNA
gccttcactggcctcagccagtcgaggg

SEQ ID NO: 24910 - DNA, 28 bp, synthetic construct
  source 1..28: mol_type = other DNA
tccctcgactggctgaggccagtgaagg

SEQ ID NO: 24911 - DNA, 28 bp, synthetic construct
  source 1..28: mol_type = other DNA
tcgtaggagctccctcgactggctgagg

SEQ ID NO: 24912 - DNA, 28 bp, synthetic construct
  source 1..28: mol_type = other DNA
tcagccagtcgagggagctcctacgagg

SEQ ID NO: 24913 - DNA, 28 bp, synthetic construct
  source 1..28: mol_type = other DNA
ataacctcgtaggagctccctcgactgg

SEQ ID NO: 24914 - DNA, 28 bp, synthetic construct
  source 1..28: mol_type = other DNA
ttgctgggctcgcagataacctcgtagg

SEQ ID NO: 24915 - DNA, 28 bp, synthetic construct
  source 1..28: mol_type = other DNA
ggttatctgcgagcccagcaaatcttgg

SEQ ID NO: 24916 - DNA, 28 bp, synthetic construct
  source 1..28: mol_type = other DNA
gttatctgcgagcccagcaaatcttggg

SEQ ID NO: 24917 - DNA, 28 bp, synthetic construct
  source 1..28: mol_type = other DNA
ttatctgcgagcccagcaaatcttgggg

SEQ ID NO: 24918 - DNA, 28 bp, synthetic construct
  source 1..28: mol_type = other DNA
tatctgcgagcccagcaaatcttggggg

SEQ ID NO: 24919 - DNA, 28 bp, synthetic construct
  source 1..28: mol_type = other DNA
ttggctaggacccccaagatttgctggg

SEQ ID NO: 24920 - DNA, 28 bp, synthetic construct
  source 1..28: mol_type = other DNA
tttggctaggacccccaagatttgctgg

SEQ ID NO: 24921 - DNA, 28 bp, synthetic construct
  source 1..28: mol_type = other DNA
agaacgttgcgcactgcatttggctagg

SEQ ID NO: 24922 - DNA, 28 bp, synthetic construct
  source 1..28: mol_type = other DNA
gagagagaacgttgcgcactgcatttgg

SEQ ID NO: 24923 - DNA, 28 bp, synthetic construct
  source 1..28: mol_type = other DNA
gcagtgcgcaacgttctctctcacttgg

SEQ ID NO: 24924 - DNA, 28 bp, synthetic construct
  source 1..28: mol_type = other DNA
gtgcgcaacgttctctctcacttggagg

SEQ ID NO: 24925 - DNA, 28 bp, synthetic construct
  source 1..28: mol_type = other DNA
ggaaaaaaaaaaacgaggtgaatggcgg

SEQ ID NO: 24926 - DNA, 28 bp, synthetic construct
  source 1..28: mol_type = other DNA
ttaggaaaaaaaaaaacgaggtgaatgg

SEQ ID NO: 24927 - DNA, 28 bp, synthetic construct
  source 1..28: mol_type = other DNA
tcacctcgtttttttttttcctaaaagg

SEQ ID NO: 24928 - DNA, 28 bp, synthetic construct
  source 1..28: mol_type = other DNA
aatccttttaggaaaaaaaaaaacgagg

SEQ ID NO: 24929 - DNA, 28 bp, synthetic construct
  source 1..28: mol_type = other DNA
agcactcagaaaaaaaaatccttttagg

SEQ ID NO: 24930 - DNA, 28 bp, synthetic construct
  source 1..28: mol_type = other DNA
aggcatgtgcaaagcaggtaaaataggg

SEQ ID NO: 24931 - DNA, 28 bp, synthetic construct
  source 1..28: mol_type = other DNA
gaggcatgtgcaaagcaggtaaaatagg

SEQ ID NO: 24932 - DNA, 28 bp, synthetic construct
  source 1..28: mol_type = other DNA
tgagggcgggaggcatgtgcaaagcagg

SEQ ID NO: 24933 - DNA, 28 bp, synthetic construct
  source 1..28: mol_type = other DNA
tttgcacatgcctcccgccctcacccgg

SEQ ID NO: 24934 - DNA, 28 bp, synthetic construct
  source 1..28: mol_type = other DNA
ttgcacatgcctcccgccctcacccggg

SEQ ID NO: 24935 - DNA, 28 bp, synthetic construct
  source 1..28: mol_type = other DNA
cacatgcctcccgccctcacccgggagg

SEQ ID NO: 24936 - DNA, 28 bp, synthetic construct
  source 1..28: mol_type = other DNA
atgcctcccgccctcacccgggaggcgg

SEQ ID NO: 24937 - DNA, 28 bp, synthetic construct
  source 1..28: mol_type = other DNA
tcgccgcctcccgggtgagggcgggagg

SEQ ID NO: 24938 - DNA, 28 bp, synthetic construct
  source 1..28: mol_type = other DNA
tcttcgccgcctcccgggtgagggcggg

SEQ ID NO: 24939 - DNA, 28 bp, synthetic construct
  source 1..28: mol_type = other DNA
gtcttcgccgcctcccgggtgagggcgg

SEQ ID NO: 24940 - DNA, 28 bp, synthetic construct
  source 1..28: mol_type = other DNA
ggcgtcttcgccgcctcccgggtgaggg

SEQ ID NO: 24941 - DNA, 28 bp, synthetic construct
  source 1..28: mol_type = other DNA
gggcgtcttcgccgcctcccgggtgagg

SEQ ID NO: 24942 - DNA, 28 bp, synthetic construct
  source 1..28: mol_type = other DNA
cccgggaggcggcgaagacgcccactgg

SEQ ID NO: 24943 - DNA, 28 bp, synthetic construct
  source 1..28: mol_type = other DNA
ccgggaggcggcgaagacgcccactggg

SEQ ID NO: 24944 - DNA, 28 bp, synthetic construct
  source 1..28: mol_type = other DNA
cgaagacgcccactgggaccgcgcctgg

SEQ ID NO: 24945 - DNA, 28 bp, synthetic construct
  source 1..28: mol_type = other DNA
gaaaacggccaggcgcggtcccagtggg

SEQ ID NO: 24946 - DNA, 28 bp, synthetic construct
  source 1..28: mol_type = other DNA
agaaaacggccaggcgcggtcccagtgg

SEQ ID NO: 24947 - DNA, 28 bp, synthetic construct
  source 1..28: mol_type = other DNA
actgggaccgcgcctggccgttttctgg

SEQ ID NO: 24948 - DNA, 28 bp, synthetic construct
  source 1..28: mol_type = other DNA
ctgggaccgcgcctggccgttttctggg

SEQ ID NO: 24949 - DNA, 28 bp, synthetic construct
  source 1..28: mol_type = other DNA
gacgcgcccagaaaacggccaggcgcgg

SEQ ID NO: 24950 - DNA, 28 bp, synthetic construct
  source 1..28: mol_type = other DNA
ggcaggacgcgcccagaaaacggccagg

SEQ ID NO: 24951 - DNA, 28 bp, synthetic construct
  source 1..28: mol_type = other DNA
gtgggggcaggacgcgcccagaaaacgg

SEQ ID NO: 24952 - DNA, 28 bp, synthetic construct
  source 1..28: mol_type = other DNA
gttttctgggcgcgtcctgcccccacgg

SEQ ID NO: 24953 - DNA, 28 bp, synthetic construct
  source 1..28: mol_type = other DNA
cctaagagacagaggccgtgggggcagg

SEQ ID NO: 24954 - DNA, 28 bp, synthetic construct
  source 1..28: mol_type = other DNA
ctgcccccacggcctctgtctcttaggg

SEQ ID NO: 24955 - DNA, 28 bp, synthetic construct
  source 1..28: mol_type = other DNA
tcgccctaagagacagaggccgtggggg

SEQ ID NO: 24956 - DNA, 28 bp, synthetic construct
  source 1..28: mol_type = other DNA
gtcgccctaagagacagaggccgtgggg

SEQ ID NO: 24957 - DNA, 28 bp, synthetic construct
  source 1..28: mol_type = other DNA
agtcgccctaagagacagaggccgtggg

SEQ ID NO: 24958 - DNA, 28 bp, synthetic construct
  source 1..28: mol_type = other DNA
cagtcgccctaagagacagaggccgtgg

SEQ ID NO: 24959 - DNA, 28 bp, synthetic construct
  source 1..28: mol_type = other DNA
cacggcctctgtctcttagggcgactgg

SEQ ID NO: 24960 - DNA, 28 bp, synthetic construct
  source 1..28: mol_type = other DNA
acggcctctgtctcttagggcgactggg

SEQ ID NO: 24961 - DNA, 28 bp, synthetic construct
  source 1..28: mol_type = other DNA
cgcgcccagtcgccctaagagacagagg

SEQ ID NO: 24962 - DNA, 28 bp, synthetic construct
  source 1..28: mol_type = other DNA
ctctgtctcttagggcgactgggcgcgg

SEQ ID NO: 24963 - DNA, 28 bp, synthetic construct
  source 1..28: mol_type = other DNA
gggcgactgggcgcggaagaaaagctgg

SEQ ID NO: 24964 - DNA, 28 bp, synthetic construct
  source 1..28: mol_type = other DNA
cggaagaaaagctggagagcccctgcgg

SEQ ID NO: 24965 - DNA, 28 bp, synthetic construct
  source 1..28: mol_type = other DNA
ggaagaaaagctggagagcccctgcggg

SEQ ID NO: 24966 - DNA, 28 bp, synthetic construct
  source 1..28: mol_type = other DNA
gaagaaaagctggagagcccctgcgggg

SEQ ID NO: 24967 - DNA, 28 bp, synthetic construct
  source 1..28: mol_type = other DNA
gaaaagctggagagcccctgcggggtgg

SEQ ID NO: 24968 - DNA, 28 bp, synthetic construct
  source 1..28: mol_type = other DNA
agctggagagcccctgcggggtggcagg

SEQ ID NO: 24969 - DNA, 28 bp, synthetic construct
  source 1..28: mol_type = other DNA
tggagagcccctgcggggtggcaggagg

SEQ ID NO: 24970 - DNA, 28 bp, synthetic construct
  source 1..28: mol_type = other DNA
agagcccctgcggggtggcaggaggagg

SEQ ID NO: 24971 - DNA, 28 bp, synthetic construct
  source 1..28: mol_type = other DNA
gagcccctgcggggtggcaggaggaggg

SEQ ID NO: 24972 - DNA, 28 bp, synthetic construct
  source 1..28: mol_type = other DNA
gcaccctcctcctgccaccccgcagggg

SEQ ID NO: 24973 - DNA, 28 bp, synthetic construct
  source 1..28: mol_type = other DNA
ggcaccctcctcctgccaccccgcaggg

SEQ ID NO: 24974 - DNA, 28 bp, synthetic construct
  source 1..28: mol_type = other DNA
aggcaccctcctcctgccaccccgcagg

SEQ ID NO: 24975 - DNA, 28 bp, synthetic construct
  source 1..28: mol_type = other DNA
gaggagggtgcctgagtcccgcgagagg

SEQ ID NO: 24976 - DNA, 28 bp, synthetic construct
  source 1..28: mol_type = other DNA
gggtgcctgagtcccgcgagaggcccgg

SEQ ID NO: 24977 - DNA, 28 bp, synthetic construct
  source 1..28: mol_type = other DNA
ggtgcctgagtcccgcgagaggcccggg

SEQ ID NO: 24978 - DNA, 28 bp, synthetic construct
  source 1..28: mol_type = other DNA
ctcgcccgggcctctcgcgggactcagg

SEQ ID NO: 24979 - DNA, 28 bp, synthetic construct
  source 1..28: mol_type = other DNA
ctgagtcccgcgagaggcccgggcgagg

SEQ ID NO: 24980 - DNA, 28 bp, synthetic construct
  source 1..28: mol_type = other DNA
catcttcctcgcccgggcctctcgcggg

SEQ ID NO: 24981 - DNA, 28 bp, synthetic construct
  source 1..28: mol_type = other DNA
gcatcttcctcgcccgggcctctcgcgg

SEQ ID NO: 24982 - DNA, 28 bp, synthetic construct
  source 1..28: mol_type = other DNA
agcaggctgcgcatcttcctcgcccggg

SEQ ID NO: 24983 - DNA, 28 bp, synthetic construct
  source 1..28: mol_type = other DNA
cagcaggctgcgcatcttcctcgcccgg

SEQ ID NO: 24984 - DNA, 28 bp, synthetic construct
  source 1..28: mol_type = other DNA
gcagcctgctgatccgcgtcccgcccgg

SEQ ID NO: 24985 - DNA, 28 bp, synthetic construct
  source 1..28: mol_type = other DNA
ggcgccgggcgggacgcggatcagcagg

SEQ ID NO: 24986 - DNA, 28 bp, synthetic construct
  source 1..28: mol_type = other DNA
gctgatccgcgtcccgcccggcgccagg

SEQ ID NO: 24987 - DNA, 28 bp, synthetic construct
  source 1..28: mol_type = other DNA
ctgatccgcgtcccgcccggcgccaggg

SEQ ID NO: 24988 - DNA, 28 bp, synthetic construct
  source 1..28: mol_type = other DNA
agggtccctggcgccgggcgggacgcgg

SEQ ID NO: 24989 - DNA, 28 bp, synthetic construct
  source 1..28: mol_type = other DNA
cctctgagggtccctggcgccgggcggg

SEQ ID NO: 24990 - DNA, 28 bp, synthetic construct
  source 1..28: mol_type = other DNA
ccgcccggcgccagggaccctcagaggg

SEQ ID NO: 24991 - DNA, 28 bp, synthetic construct
  source 1..28: mol_type = other DNA
cctccctctgagggtccctggcgccggg

SEQ ID NO: 24992 - DNA, 28 bp, synthetic construct
  source 1..28: mol_type = other DNA
tcctccctctgagggtccctggcgccgg

SEQ ID NO: 24993 - DNA, 28 bp, synthetic construct
  source 1..28: mol_type = other DNA
gagctctcctccctctgagggtccctgg

SEQ ID NO: 24994 - DNA, 28 bp, synthetic construct
  source 1..28: mol_type = other DNA
ggtctttgagctctcctccctctgaggg

SEQ ID NO: 24995 - DNA, 28 bp, synthetic construct
  source 1..28: mol_type = other DNA
aggtctttgagctctcctccctctgagg

SEQ ID NO: 24996 - DNA, 28 bp, synthetic construct
  source 1..28: mol_type = other DNA
aaagacctcgccccgcgccttcgcgagg

SEQ ID NO: 24997 - DNA, 28 bp, synthetic construct
  source 1..28: mol_type = other DNA
ttggtcctcgcgaaggcgcggggcgagg

SEQ ID NO: 24998 - DNA, 28 bp, synthetic construct
  source 1..28: mol_type = other DNA
ctgggttggtcctcgcgaaggcgcgggg

SEQ ID NO: 24999 - DNA, 28 bp, synthetic construct
  source 1..28: mol_type = other DNA
actgggttggtcctcgcgaaggcgcggg

SEQ ID NO: 25000 - DNA, 28 bp, synthetic construct
  source 1..28: mol_type = other DNA
gactgggttggtcctcgcgaaggcgcgg

SEQ ID NO: 25001 - DNA, 28 bp, synthetic construct
  source 1..28: mol_type = other DNA
gcggggactgggttggtcctcgcgaagg

SEQ ID NO: 25002 - DNA, 28 bp, synthetic construct
  source 1..28: mol_type = other DNA
tctggggcaggcgcggggactgggttgg

SEQ ID NO: 25003 - DNA, 28 bp, synthetic construct
  source 1..28: mol_type = other DNA
cccagtccccgcgcctgccccagagcgg

SEQ ID NO: 25004 - DNA, 28 bp, synthetic construct
  source 1..28: mol_type = other DNA
gccgctctggggcaggcgcggggactgg

SEQ ID NO: 25005 - DNA, 28 bp, synthetic construct
  source 1..28: mol_type = other DNA
tctaagccgctctggggcaggcgcgggg

SEQ ID NO: 25006 - DNA, 28 bp, synthetic construct
  source 1..28: mol_type = other DNA
ttctaagccgctctggggcaggcgcggg

SEQ ID NO: 25007 - DNA, 28 bp, synthetic construct
  source 1..28: mol_type = other DNA
tttctaagccgctctggggcaggcgcgg

SEQ ID NO: 25008 - DNA, 28 bp, synthetic construct
  source 1..28: mol_type = other DNA
ctgagtttctaagccgctctggggcagg

SEQ ID NO: 25009 - DNA, 28 bp, synthetic construct
  source 1..28: mol_type = other DNA
ctgccccagagcggcttagaaactcagg

SEQ ID NO: 25010 - DNA, 28 bp, synthetic construct
  source 1..28: mol_type = other DNA
tgccccagagcggcttagaaactcaggg

SEQ ID NO: 25011 - DNA, 28 bp, synthetic construct
  source 1..28: mol_type = other DNA
tgccctgagtttctaagccgctctgggg

SEQ ID NO: 25012 - DNA, 28 bp, synthetic construct
  source 1..28: mol_type = other DNA
gtgccctgagtttctaagccgctctggg

SEQ ID NO: 25013 - DNA, 28 bp, synthetic construct
  source 1..28: mol_type = other DNA
tgtgccctgagtttctaagccgctctgg

SEQ ID NO: 25014 - DNA, 28 bp, synthetic construct
  source 1..28: mol_type = other DNA
gaaactcagggcacagtgagagcgcagg

SEQ ID NO: 25015 - DNA, 28 bp, synthetic construct
  source 1..28: mol_type = other DNA
aaactcagggcacagtgagagcgcaggg

SEQ ID NO: 25016 - DNA, 28 bp, synthetic construct
  source 1..28: mol_type = other DNA
cagtgagagcgcagggcgcctcccgagg

SEQ ID NO: 25017 - DNA, 28 bp, synthetic construct
  source 1..28: mol_type = other DNA
ggcgcctcccgaggcttcacaccgccgg

SEQ ID NO: 25018 - DNA, 28 bp, synthetic construct
  source 1..28: mol_type = other DNA
ccggccggcggtgtgaagcctcgggagg

SEQ ID NO: 25019 - DNA, 28 bp, synthetic construct
  source 1..28: mol_type = other DNA
ctcccgaggcttcacaccgccggccggg

SEQ ID NO: 25020 - DNA, 28 bp, synthetic construct
  source 1..28: mol_type = other DNA
ggcccggccggcggtgtgaagcctcggg

SEQ ID NO: 25021 - DNA, 28 bp, synthetic construct
  source 1..28: mol_type = other DNA
tggcccggccggcggtgtgaagcctcgg

SEQ ID NO: 25022 - DNA, 28 bp, synthetic construct
  source 1..28: mol_type = other DNA
ggcttcacaccgccggccgggccagcgg

SEQ ID NO: 25023 - DNA, 28 bp, synthetic construct
  source 1..28: mol_type = other DNA
ttcacaccgccggccgggccagcggagg

SEQ ID NO: 25024 - DNA, 28 bp, synthetic construct
  source 1..28: mol_type = other DNA
tcacagcctccgctggcccggccggcgg

SEQ ID NO: 25025 - DNA, 28 bp, synthetic construct
  source 1..28: mol_type = other DNA
cggtcacagcctccgctggcccggccgg

SEQ ID NO: 25026 - DNA, 28 bp, synthetic construct
  source 1..28: mol_type = other DNA
cggccgggccagcggaggctgtgaccgg

SEQ ID NO: 25027 - DNA, 28 bp, synthetic construct
  source 1..28: mol_type = other DNA
gctccggtcacagcctccgctggcccgg

SEQ ID NO: 25028 - DNA, 28 bp, synthetic construct
  source 1..28: mol_type = other DNA
ggggcgctccggtcacagcctccgctgg

SEQ ID NO: 25029 - DNA, 28 bp, synthetic construct
  source 1..28: mol_type = other DNA
cgtgcgcggcacagagggggcgctccgg

SEQ ID NO: 25030 - DNA, 28 bp, synthetic construct
  source 1..28: mol_type = other DNA
cgccccctctgtgccgcgcacgccgcgg

SEQ ID NO: 25031 - DNA, 28 bp, synthetic construct
  source 1..28: mol_type = other DNA
ggccgcggcgtgcgcggcacagaggggg

SEQ ID NO: 25032 - DNA, 28 bp, synthetic construct
  source 1..28: mol_type = other DNA
cggccgcggcgtgcgcggcacagagggg

SEQ ID NO: 25033 - DNA, 28 bp, synthetic construct
  source 1..28: mol_type = other DNA
gcggccgcggcgtgcgcggcacagaggg

SEQ ID NO: 25034 - DNA, 28 bp, synthetic construct
  source 1..28: mol_type = other DNA
ggcggccgcggcgtgcgcggcacagagg

SEQ ID NO: 25035 - DNA, 28 bp, synthetic construct
  source 1..28: mol_type = other DNA
gtgccgcgcacgccgcggccgccgccgg

SEQ ID NO: 25036 - DNA, 28 bp, synthetic construct
  source 1..28: mol_type = other DNA
tgccgcgcacgccgcggccgccgccggg

SEQ ID NO: 25037 - DNA, 28 bp, synthetic construct
  source 1..28: mol_type = other DNA
aacccggcggcggccgcggcgtgcgcgg

SEQ ID NO: 25038 - DNA, 28 bp, synthetic construct
  source 1..28: mol_type = other DNA
gcgcacgccgcggccgccgccgggttgg

SEQ ID NO: 25039 - DNA, 28 bp, synthetic construct
  source 1..28: mol_type = other DNA
cgcacgccgcggccgccgccgggttggg

SEQ ID NO: 25040 - DNA, 28 bp, synthetic construct
  source 1..28: mol_type = other DNA
gcacgccgcggccgccgccgggttgggg

SEQ ID NO: 25041 - DNA, 28 bp, synthetic construct
  source 1..28: mol_type = other DNA
gccgcggccgccgccgggttggggtagg

SEQ ID NO: 25042 - DNA, 28 bp, synthetic construct
  source 1..28: mol_type = other DNA
acctaccccaacccggcggcggccgcgg

SEQ ID NO: 25043 - DNA, 28 bp, synthetic construct
  source 1..28: mol_type = other DNA
ccgccgccgggttggggtaggtgagcgg

SEQ ID NO: 25044 - DNA, 28 bp, synthetic construct
  source 1..28: mol_type = other DNA
cgccgccgggttggggtaggtgagcggg

SEQ ID NO: 25045 - DNA, 28 bp, synthetic construct
  source 1..28: mol_type = other DNA
ctcccgctcacctaccccaacccggcgg

SEQ ID NO: 25046 - DNA, 28 bp, synthetic construct
  source 1..28: mol_type = other DNA
cgccgggttggggtaggtgagcgggagg

SEQ ID NO: 25047 - DNA, 28 bp, synthetic construct
  source 1..28: mol_type = other DNA
agcctcccgctcacctaccccaacccgg

SEQ ID NO: 25048 - DNA, 28 bp, synthetic construct
  source 1..28: mol_type = other DNA
ggttggggtaggtgagcgggaggctagg

SEQ ID NO: 25049 - DNA, 28 bp, synthetic construct
  source 1..28: mol_type = other DNA
gttggggtaggtgagcgggaggctaggg

SEQ ID NO: 25050 - DNA, 28 bp, synthetic construct
  source 1..28: mol_type = other DNA
gtgagcgggaggctagggtacacttcgg

SEQ ID NO: 25051 - DNA, 28 bp, synthetic construct
  source 1..28: mol_type = other DNA
tgagcgggaggctagggtacacttcggg

SEQ ID NO: 25052 - DNA, 28 bp, synthetic construct
  source 1..28: mol_type = other DNA
gagcgggaggctagggtacacttcgggg

SEQ ID NO: 25053 - DNA, 28 bp, synthetic construct
  source 1..28: mol_type = other DNA
cgggaggctagggtacacttcggggtgg

SEQ ID NO: 25054 - DNA, 28 bp, synthetic construct
  source 1..28: mol_type = other DNA
gggaggctagggtacacttcggggtggg

SEQ ID NO: 25055 - DNA, 28 bp, synthetic construct
  source 1..28: mol_type = other DNA
ggaggctagggtacacttcggggtgggg

SEQ ID NO: 25056 - DNA, 28 bp, synthetic construct
  source 1..28: mol_type = other DNA
gaggctagggtacacttcggggtggggg

SEQ ID NO: 25057 - DNA, 28 bp, synthetic construct
  source 1..28: mol_type = other DNA
ctagggtacacttcggggtgggggatgg

SEQ ID NO: 25058 - DNA, 28 bp, synthetic construct
  source 1..28: mol_type = other DNA
tagggtacacttcggggtgggggatggg

SEQ ID NO: 25059 - DNA, 28 bp, synthetic construct
  source 1..28: mol_type = other DNA
tcggggtgggggatgggcgcgcacatgg

SEQ ID NO: 25060 - DNA, 28 bp, synthetic construct
  source 1..28: mol_type = other DNA
gatgggcgcgcacatggccgccagcagg

SEQ ID NO: 25061 - DNA, 28 bp, synthetic construct
  source 1..28: mol_type = other DNA
tggccgccagcaggcagagttactccgg

SEQ ID NO: 25062 - DNA, 28 bp, synthetic construct
  source 1..28: mol_type = other DNA
ttaccggagtaactctgcctgctggcgg

SEQ ID NO: 25063 - DNA, 28 bp, synthetic construct
  source 1..28: mol_type = other DNA
tgtttaccggagtaactctgcctgctgg

SEQ ID NO: 25064 - DNA, 28 bp, synthetic construct
  source 1..28: mol_type = other DNA
gcagagttactccggtaaacacgccagg

SEQ ID NO: 25065 - DNA, 28 bp, synthetic construct
  source 1..28: mol_type = other DNA
cagagttactccggtaaacacgccaggg

SEQ ID NO: 25066 - DNA, 28 bp, synthetic construct
  source 1..28: mol_type = other DNA
gttactccggtaaacacgccagggacgg

SEQ ID NO: 25067 - DNA, 28 bp, synthetic construct
  source 1..28: mol_type = other DNA
actccggtaaacacgccagggacggcgg

SEQ ID NO: 25068 - DNA, 28 bp, synthetic construct
  source 1..28: mol_type = other DNA
gcgccgccgtccctggcgtgtttaccgg

SEQ ID NO: 25069 - DNA, 28 bp, synthetic construct
  source 1..28: mol_type = other DNA
aacacgccagggacggcggcgcgcgcgg

SEQ ID NO: 25070 - DNA, 28 bp, synthetic construct
  source 1..28: mol_type = other DNA
acacgccagggacggcggcgcgcgcggg

SEQ ID NO: 25071 - DNA, 28 bp, synthetic construct
  source 1..28: mol_type = other DNA
cgccagggacggcggcgcgcgcgggagg

SEQ ID NO: 25072 - DNA, 28 bp, synthetic construct
  source 1..28: mol_type = other DNA
tgcctcccgcgcgcgccgccgtccctgg

SEQ ID NO: 25073 - DNA, 28 bp, synthetic construct
  source 1..28: mol_type = other DNA
gcggcgcgcgcgggaggcaacccagcgg

SEQ ID NO: 25074 - DNA, 28 bp, synthetic construct
  source 1..28: mol_type = other DNA
cggcgcgcgcgggaggcaacccagcggg

SEQ ID NO: 25075 - DNA, 28 bp, synthetic construct
  source 1..28: mol_type = other DNA
ggcgcgcgcgggaggcaacccagcgggg

SEQ ID NO: 25076 - DNA, 28 bp, synthetic construct
  source 1..28: mol_type = other DNA
aggtaaaggcgggggttgccccgctggg

SEQ ID NO: 25077 - DNA, 28 bp, synthetic construct
  source 1..28: mol_type = other DNA
caggtaaaggcgggggttgccccgctgg

SEQ ID NO: 25078 - DNA, 28 bp, synthetic construct
  source 1..28: mol_type = other DNA
tgcaggctcggacaggtaaaggcggggg

SEQ ID NO: 25079 - DNA, 28 bp, synthetic construct
  source 1..28: mol_type = other DNA
gtgcaggctcggacaggtaaaggcgggg

SEQ ID NO: 25080 - DNA, 28 bp, synthetic construct
  source 1..28: mol_type = other DNA
cgtgcaggctcggacaggtaaaggcggg

SEQ ID NO: 25081 - DNA, 28 bp, synthetic construct
  source 1..28: mol_type = other DNA
gcgtgcaggctcggacaggtaaaggcgg

SEQ ID NO: 25082 - DNA, 28 bp, synthetic construct
  source 1..28: mol_type = other DNA
ggcgcgtgcaggctcggacaggtaaagg

SEQ ID NO: 25083 - DNA, 28 bp, synthetic construct
  source 1..28: mol_type = other DNA
tttacctgtccgagcctgcacgcgccgg

SEQ ID NO: 25084 - DNA, 28 bp, synthetic construct
  source 1..28: mol_type = other DNA
acctgtccgagcctgcacgcgccggcgg

SEQ ID NO: 25085 - DNA, 28 bp, synthetic construct
  source 1..28: mol_type = other DNA
gccgccggcgcgtgcaggctcggacagg

SEQ ID NO: 25086 - DNA, 28 bp, synthetic construct
  source 1..28: mol_type = other DNA
ccgagcctgcacgcgccggcggccgcgg

SEQ ID NO: 25087 - DNA, 28 bp, synthetic construct
  source 1..28: mol_type = other DNA
cggcgccgcggccgccggcgcgtgcagg

SEQ ID NO: 25088 - DNA, 28 bp, synthetic construct
  source 1..28: mol_type = other DNA
gcacgcgccggcggccgcggcgccgagg

SEQ ID NO: 25089 - DNA, 28 bp, synthetic construct
  source 1..28: mol_type = other DNA
cacgcgccggcggccgcggcgccgaggg

SEQ ID NO: 25090 - DNA, 28 bp, synthetic construct
  source 1..28: mol_type = other DNA
acgcgccggcggccgcggcgccgagggg

SEQ ID NO: 25091 - DNA, 28 bp, synthetic construct
  source 1..28: mol_type = other DNA
cgcgccggcggccgcggcgccgaggggg

SEQ ID NO: 25092 - DNA, 28 bp, synthetic construct
  source 1..28: mol_type = other DNA
gcgccggcggccgcggcgccgagggggg

SEQ ID NO: 25093 - DNA, 28 bp, synthetic construct
  source 1..28: mol_type = other DNA
ccggcggccgcggcgccgaggggggcgg

SEQ ID NO: 25094 - DNA, 28 bp, synthetic construct
  source 1..28: mol_type = other DNA
gcaagctccgcccccctcggcgccgcgg

SEQ ID NO: 25095 - DNA, 28 bp, synthetic construct
  source 1..28: mol_type = other DNA
gcgggctggcaagctccgcccccctcgg

SEQ ID NO: 25096 - DNA, 28 bp, synthetic construct
  source 1..28: mol_type = other DNA
gggcggagcttgccagcccgcgcgccgg

SEQ ID NO: 25097 - DNA, 28 bp, synthetic construct
  source 1..28: mol_type = other DNA
ggcggagcttgccagcccgcgcgccggg

SEQ ID NO: 25098 - DNA, 28 bp, synthetic construct
  source 1..28: mol_type = other DNA
gcggagcttgccagcccgcgcgccgggg

SEQ ID NO: 25099 - DNA, 28 bp, synthetic construct
  source 1..28: mol_type = other DNA
gagcttgccagcccgcgcgccggggcgg

SEQ ID NO: 25100 - DNA, 28 bp, synthetic construct
  source 1..28: mol_type = other DNA
agcttgccagcccgcgcgccggggcggg

SEQ ID NO: 25101 - DNA, 28 bp, synthetic construct
  source 1..28: mol_type = other DNA
ctaggtcccgccccggcgcgcgggctgg

SEQ ID NO: 25102 - DNA, 28 bp, synthetic construct
  source 1..28: mol_type = other DNA
gcccgcgcgccggggcgggacctagcgg

SEQ ID NO: 25103 - DNA, 28 bp, synthetic construct
  source 1..28: mol_type = other DNA
cccgcgcgccggggcgggacctagcggg

SEQ ID NO: 25104 - DNA, 28 bp, synthetic construct
  source 1..28: mol_type = other DNA
ccgcgcgccggggcgggacctagcgggg

SEQ ID NO: 25105 - DNA, 28 bp, synthetic construct
  source 1..28: mol_type = other DNA
cgcgcgccggggcgggacctagcggggg

SEQ ID NO: 25106 - DNA, 28 bp, synthetic construct
  source 1..28: mol_type = other DNA
gcgccggggcgggacctagcgggggcgg

SEQ ID NO: 25107 - DNA, 28 bp, synthetic construct
  source 1..28: mol_type = other DNA
cgccggggcgggacctagcgggggcggg

SEQ ID NO: 25108 - DNA, 28 bp, synthetic construct
  source 1..28: mol_type = other DNA
gccggggcgggacctagcgggggcgggg

SEQ ID NO: 25109 - DNA, 28 bp, synthetic construct
  source 1..28: mol_type = other DNA
accccgcccccgctaggtcccgccccgg

SEQ ID NO: 25110 - DNA, 28 bp, synthetic construct
  source 1..28: mol_type = other DNA
aatcactgcggaccccgcccccgctagg

SEQ ID NO: 25111 - DNA, 28 bp, synthetic construct
  source 1..28: mol_type = other DNA
tagcgggggcggggtccgcagtgattgg

SEQ ID NO: 25112 - DNA, 28 bp, synthetic construct
  source 1..28: mol_type = other DNA
agcgggggcggggtccgcagtgattggg

SEQ ID NO: 25113 - DNA, 28 bp, synthetic construct
  source 1..28: mol_type = other DNA
ggcggggtccgcagtgattgggcgtagg

SEQ ID NO: 25114 - DNA, 28 bp, synthetic construct
  source 1..28: mol_type = other DNA
ggtccgcagtgattgggcgtaggagcgg

SEQ ID NO: 25115 - DNA, 28 bp, synthetic construct
  source 1..28: mol_type = other DNA
gtccgcagtgattgggcgtaggagcggg

SEQ ID NO: 25116 - DNA, 28 bp, synthetic construct
  source 1..28: mol_type = other DNA
tccgcagtgattgggcgtaggagcgggg

SEQ ID NO: 25117 - DNA, 28 bp, synthetic construct
  source 1..28: mol_type = other DNA
gccccgctcctacgcccaatcactgcgg

SEQ ID NO: 25118 - DNA, 28 bp, synthetic construct
  source 1..28: mol_type = other DNA
taggagcggggccgccagccagagctgg

SEQ ID NO: 25119 - DNA, 28 bp, synthetic construct
  source 1..28: mol_type = other DNA
aggagcggggccgccagccagagctggg

SEQ ID NO: 25120 - DNA, 28 bp, synthetic construct
  source 1..28: mol_type = other DNA
gggccgccagccagagctgggctgcagg

SEQ ID NO: 25121 - DNA, 28 bp, synthetic construct
  source 1..28: mol_type = other DNA
ggccgccagccagagctgggctgcaggg

SEQ ID NO: 25122 - DNA, 28 bp, synthetic construct
  source 1..28: mol_type = other DNA
ggccctgcagcccagctctggctggcgg

SEQ ID NO: 25123 - DNA, 28 bp, synthetic construct
  source 1..28: mol_type = other DNA
cgcggccctgcagcccagctctggctgg

SEQ ID NO: 25124 - DNA, 28 bp, synthetic construct
  source 1..28: mol_type = other DNA
ccagagctgggctgcagggccgcgcagg

SEQ ID NO: 25125 - DNA, 28 bp, synthetic construct
  source 1..28: mol_type = other DNA
tgcgcggagcgaagtgaaacctgcgcgg

SEQ ID NO: 25126 - DNA, 28 bp, synthetic construct
  source 1..28: mol_type = other DNA
tttcacttcgctccgcgcagccgcctgg

SEQ ID NO: 25127 - DNA, 28 bp, synthetic construct
  source 1..28: mol_type = other DNA
acaaactgcagaccaggcggctgcgcgg

SEQ ID NO: 25128 - DNA, 28 bp, synthetic construct
  source 1..28: mol_type = other DNA
cgcagccgcctggtctgcagtttgttgg

SEQ ID NO: 25129 - DNA, 28 bp, synthetic construct
  source 1..28: mol_type = other DNA
gagctccaacaaactgcagaccaggcgg

SEQ ID NO: 25130 - DNA, 28 bp, synthetic construct
  source 1..28: mol_type = other DNA
gcagagctccaacaaactgcagaccagg

SEQ ID NO: 25131 - DNA, 28 bp, synthetic construct
  source 1..28: mol_type = other DNA
gcggcggcggcagcggcagcggcgctgg

SEQ ID NO: 25132 - DNA, 28 bp, synthetic construct
  source 1..28: mol_type = other DNA
gcggcggcggcggcggcagcggcagcgg

SEQ ID NO: 25133 - DNA, 28 bp, synthetic construct
  source 1..28: mol_type = other DNA
gcggcggcggcggcggcggcggcagcgg

SEQ ID NO: 25134 - DNA, 28 bp, synthetic construct
  source 1..28: mol_type = other DNA
gcggcggcggcggcggcggcggcggcgg

SEQ ID NO: 25135 - DNA, 28 bp, synthetic construct
  source 1..28: mol_type = other DNA
gcggcggcggcggcggcggcggcggcgg

SEQ ID NO: 25136 - DNA, 28 bp, synthetic construct
  source 1..28: mol_type = other DNA
gcggcggcggcggcggcggcggcggcgg

SEQ ID NO: 25137 - DNA, 28 bp, synthetic construct
  source 1..28: mol_type = other DNA
gcggcggcggcggcggcggcggcggcgg

SEQ ID NO: 25138 - DNA, 28 bp, synthetic construct
  source 1..28: mol_type = other DNA
gcggcggcggcggcggcggcggcggcgg

SEQ ID NO: 25139 - DNA, 28 bp, synthetic construct
  source 1..28: mol_type = other DNA
gtggcggcggcggcggcggcggcggcgg

SEQ ID NO: 25140 - DNA, 28 bp, synthetic construct
  source 1..28: mol_type = other DNA
gtagtggcggcggcggcggcggcggcgg

SEQ ID NO: 25141 - DNA, 28 bp, synthetic construct
  source 1..28: mol_type = other DNA
gtggtagtggcggcggcggcggcggcgg

SEQ ID NO: 25142 - DNA, 28 bp, synthetic construct
  source 1..28: mol_type = other DNA
gtggtggtagtggcggcggcggcggcgg

SEQ ID NO: 25143 - DNA, 28 bp, synthetic construct
  source 1..28: mol_type = other DNA
caagtggtggtagtggcggcggcggcgg

SEQ ID NO: 25144 - DNA, 28 bp, synthetic construct
  source 1..28: mol_type = other DNA
aatcaagtggtggtagtggcggcggcgg

SEQ ID NO: 25145 - DNA, 28 bp, synthetic construct
  source 1..28: mol_type = other DNA
aagaatcaagtggtggtagtggcggcgg

SEQ ID NO: 25146 - DNA, 28 bp, synthetic construct
  source 1..28: mol_type = other DNA
tgcaagaatcaagtggtggtagtggcgg

SEQ ID NO: 25147 - DNA, 28 bp, synthetic construct
  source 1..28: mol_type = other DNA
ggctgcaagaatcaagtggtggtagtgg

SEQ ID NO: 25148 - DNA, 28 bp, synthetic construct
  source 1..28: mol_type = other DNA
cagggtggctgcaagaatcaagtggtgg

SEQ ID NO: 25149 - DNA, 28 bp, synthetic construct
  source 1..28: mol_type = other DNA
tcgcagggtggctgcaagaatcaagtgg

SEQ ID NO: 25150 - DNA, 28 bp, synthetic construct
  source 1..28: mol_type = other DNA
tcgcagtgtggcagggttcgcagggtgg

SEQ ID NO: 25151 - DNA, 28 bp, synthetic construct
  source 1..28: mol_type = other DNA
cgatcgcagtgtggcagggttcgcaggg

SEQ ID NO: 25152 - DNA, 28 bp, synthetic construct
  source 1..28: mol_type = other DNA
gcgatcgcagtgtggcagggttcgcagg

SEQ ID NO: 25153 - DNA, 28 bp, synthetic construct
  source 1..28: mol_type = other DNA
gcgatgatgcgatcgcagtgtggcaggg

SEQ ID NO: 25154 - DNA, 28 bp, synthetic construct
  source 1..28: mol_type = other DNA
cgcgatgatgcgatcgcagtgtggcagg

SEQ ID NO: 25155 - DNA, 28 bp, synthetic construct
  source 1..28: mol_type = other DNA
ctgccacactgcgatcgcatcatcgcgg

SEQ ID NO: 25156 - DNA, 28 bp, synthetic construct
  source 1..28: mol_type = other DNA
ataccgcgatgatgcgatcgcagtgtgg

SEQ ID NO: 25157 - DNA, 28 bp, synthetic construct
  source 1..28: mol_type = other DNA
actgcgatcgcatcatcgcggtattcgg

SEQ ID NO: 25158 - DNA, 28 bp, synthetic construct
  source 1..28: mol_type = other DNA
cgctgcgttcccgccgccaccgcctcgg

SEQ ID NO: 25159 - DNA, 28 bp, synthetic construct
  source 1..28: mol_type = other DNA
gaaagggcgccgaggcggtggcggcggg

SEQ ID NO: 25160 - DNA, 28 bp, synthetic construct
  source 1..28: mol_type = other DNA
agaaagggcgccgaggcggtggcggcgg

SEQ ID NO: 25161 - DNA, 28 bp, synthetic construct
  source 1..28: mol_type = other DNA
ccaagaaagggcgccgaggcggtggcgg

SEQ ID NO: 25162 - DNA, 28 bp, synthetic construct
  source 1..28: mol_type = other DNA
gggccaagaaagggcgccgaggcggtgg

SEQ ID NO: 25163 - DNA, 28 bp, synthetic construct
  source 1..28: mol_type = other DNA
caagggccaagaaagggcgccgaggcgg

SEQ ID NO: 25164 - DNA, 28 bp, synthetic construct
  source 1..28: mol_type = other DNA
gaacaagggccaagaaagggcgccgagg

SEQ ID NO: 25165 - DNA, 28 bp, synthetic construct
  source 1..28: mol_type = other DNA
atttgggggaacaagggccaagaaaggg

SEQ ID NO: 25166 - DNA, 28 bp, synthetic construct
  source 1..28: mol_type = other DNA
catttgggggaacaagggccaagaaagg

SEQ ID NO: 25167 - DNA, 28 bp, synthetic construct
  source 1..28: mol_type = other DNA
cagagtcagacatttgggggaacaaggg

SEQ ID NO: 25168 - DNA, 28 bp, synthetic construct
  source 1..28: mol_type = other DNA
tcagagtcagacatttgggggaacaagg

SEQ ID NO: 25169 - DNA, 28 bp, synthetic construct
  source 1..28: mol_type = other DNA
cccccaaatgtctgactctgactctcgg

SEQ ID NO: 25170 - DNA, 28 bp, synthetic construct
  source 1..28: mol_type = other DNA
tccgagagtcagagtcagacatttgggg

SEQ ID NO: 25171 - DNA, 28 bp, synthetic construct
  source 1..28: mol_type = other DNA
gtccgagagtcagagtcagacatttggg

SEQ ID NO: 25172 - DNA, 28 bp, synthetic construct
  source 1..28: mol_type = other DNA
agtccgagagtcagagtcagacatttgg

SEQ ID NO: 25173 - DNA, 28 bp, synthetic construct
  source 1..28: mol_type = other DNA
tctgactctcggactgagaaacgcaagg

SEQ ID NO: 25174 - DNA, 28 bp, synthetic construct
  source 1..28: mol_type = other DNA
acgcaaggtaaatacctccaaatcccgg

SEQ ID NO: 25175 - DNA, 28 bp, synthetic construct
  source 1..28: mol_type = other DNA
cgcaaggtaaatacctccaaatcccggg

SEQ ID NO: 25176 - DNA, 28 bp, synthetic construct
  source 1..28: mol_type = other DNA
gcaaggtaaatacctccaaatcccgggg

SEQ ID NO: 25177 - DNA, 28 bp, synthetic construct
  source 1..28: mol_type = other DNA
gtaaatacctccaaatcccggggcgcgg

SEQ ID NO: 25178 - DNA, 28 bp, synthetic construct
  source 1..28: mol_type = other DNA
taaatacctccaaatcccggggcgcggg

SEQ ID NO: 25179 - DNA, 28 bp, synthetic construct
  source 1..28: mol_type = other DNA
acctccaaatcccggggcgcgggcctgg

SEQ ID NO: 25180 - DNA, 28 bp, synthetic construct
  source 1..28: mol_type = other DNA
gccaggcccgcgccccgggatttggagg

SEQ ID NO: 25181 - DNA, 28 bp, synthetic construct
  source 1..28: mol_type = other DNA
ggtgccaggcccgcgccccgggatttgg

SEQ ID NO: 25182 - DNA, 28 bp, synthetic construct
  source 1..28: mol_type = other DNA
tcccggggcgcgggcctggcaccgaagg

SEQ ID NO: 25183 - DNA, 28 bp, synthetic construct
  source 1..28: mol_type = other DNA
tccttcggtgccaggcccgcgccccggg

SEQ ID NO: 25184 - DNA, 28 bp, synthetic construct
  source 1..28: mol_type = other DNA
ttccttcggtgccaggcccgcgccccgg

SEQ ID NO: 25185 - DNA, 28 bp, synthetic construct
  source 1..28: mol_type = other DNA
ccagcgctagtcttccttcggtgccagg

SEQ ID NO: 25186 - DNA, 28 bp, synthetic construct
  source 1..28: mol_type = other DNA
tcgggctccagcgctagtcttccttcgg

SEQ ID NO: 25187 - DNA, 28 bp, synthetic construct
  source 1..28: mol_type = other DNA
aggaagactagcgctggagcccgaacgg

SEQ ID NO: 25188 - DNA, 28 bp, synthetic construct
  source 1..28: mol_type = other DNA
aagcgggcagtaggtggtgccgttcggg

SEQ ID NO: 25189 - DNA, 28 bp, synthetic construct
  source 1..28: mol_type = other DNA
gaagcgggcagtaggtggtgccgttcgg

SEQ ID NO: 25190 - DNA, 28 bp, synthetic construct
  source 1..28: mol_type = other DNA
acgtgcacgggaagcgggcagtaggtgg

SEQ ID NO: 25191 - DNA, 28 bp, synthetic construct
  source 1..28: mol_type = other DNA
cgcacgtgcacgggaagcgggcagtagg

SEQ ID NO: 25192 - DNA, 28 bp, synthetic construct
  source 1..28: mol_type = other DNA
tgcccgcttcccgtgcacgtgcgagcgg

SEQ ID NO: 25193 - DNA, 28 bp, synthetic construct
  source 1..28: mol_type = other DNA
ctccgctcgcacgtgcacgggaagcggg

SEQ ID NO: 25194 - DNA, 28 bp, synthetic construct
  source 1..28: mol_type = other DNA
tctccgctcgcacgtgcacgggaagcgg

SEQ ID NO: 25195 - DNA, 28 bp, synthetic construct
  source 1..28: mol_type = other DNA
caagcgtctccgctcgcacgtgcacggg

SEQ ID NO: 25196 - DNA, 28 bp, synthetic construct
  source 1..28: mol_type = other DNA
gcaagcgtctccgctcgcacgtgcacgg

SEQ ID NO: 25197 - DNA, 28 bp, synthetic construct
  source 1..28: mol_type = other DNA
cacgtgcgagcggagacgcttgcatcgg

SEQ ID NO: 25198 - DNA, 28 bp, synthetic construct
  source 1..28: mol_type = other DNA
cgcttgcatcggcgccgcttgtcgccgg

SEQ ID NO: 25199 - DNA, 28 bp, synthetic construct
  source 1..28: mol_type = other DNA
ttgcatcggcgccgcttgtcgccggcgg

SEQ ID NO: 25200 - DNA, 28 bp, synthetic construct
  source 1..28: mol_type = other DNA
tgcatcggcgccgcttgtcgccggcggg

SEQ ID NO: 25201 - DNA, 28 bp, synthetic construct
  source 1..28: mol_type = other DNA
atcggcgccgcttgtcgccggcgggagg

SEQ ID NO: 25202 - DNA, 28 bp, synthetic construct
  source 1..28: mol_type = other DNA
ggcgccgcttgtcgccggcgggaggtgg

SEQ ID NO: 25203 - DNA, 28 bp, synthetic construct
  source 1..28: mol_type = other DNA
gcgccgcttgtcgccggcgggaggtggg

SEQ ID NO: 25204 - DNA, 28 bp, synthetic construct
  source 1..28: mol_type = other DNA
cgccgcttgtcgccggcgggaggtgggg

SEQ ID NO: 25205 - DNA, 28 bp, synthetic construct
  source 1..28: mol_type = other DNA
atccccacctcccgccggcgacaagcgg

SEQ ID NO: 25206 - DNA, 28 bp, synthetic construct
  source 1..28: mol_type = other DNA
cgccggcgggaggtggggatccgtgtgg

SEQ ID NO: 25207 - DNA, 28 bp, synthetic construct
  source 1..28: mol_type = other DNA
atccacacggatccccacctcccgccgg

SEQ ID NO: 25208 - DNA, 28 bp, synthetic construct
  source 1..28: mol_type = other DNA
gcgggaggtggggatccgtgtggatcgg

SEQ ID NO: 25209 - DNA, 28 bp, synthetic construct
  source 1..28: mol_type = other DNA
cgggaggtggggatccgtgtggatcggg

SEQ ID NO: 25210 - DNA, 28 bp, synthetic construct
  source 1..28: mol_type = other DNA
gatccgtgtggatcgggttccctctcgg

SEQ ID NO: 25211 - DNA, 28 bp, synthetic construct
  source 1..28: mol_type = other DNA
atccgtgtggatcgggttccctctcggg

SEQ ID NO: 25212 - DNA, 28 bp, synthetic construct
  source 1..28: mol_type = other DNA
tgcccgagagggaacccgatccacacgg

SEQ ID NO: 25213 - DNA, 28 bp, synthetic construct
  source 1..28: mol_type = other DNA
gtgtggatcgggttccctctcgggcagg

SEQ ID NO: 25214 - DNA, 28 bp, synthetic construct
  source 1..28: mol_type = other DNA
ttctttaaagagaacctgcccgagaggg

SEQ ID NO: 25215 - DNA, 28 bp, synthetic construct
  source 1..28: mol_type = other DNA
tttctttaaagagaacctgcccgagagg

SEQ ID NO: 25216 - DNA, 28 bp, synthetic construct
  source 1..28: mol_type = other DNA
tctctttaaagaaaagtcgttcacgcgg

SEQ ID NO: 25217 - DNA, 28 bp, synthetic construct
  source 1..28: mol_type = other DNA
gaaaagtcgttcacgcggaacctgcagg

SEQ ID NO: 25218 - DNA, 28 bp, synthetic construct
  source 1..28: mol_type = other DNA
cgttcacgcggaacctgcaggctcttgg

SEQ ID NO: 25219 - DNA, 28 bp, synthetic construct
  source 1..28: mol_type = other DNA
aacctgcaggctcttggccgaagtgcgg

SEQ ID NO: 25220 - DNA, 28 bp, synthetic construct
  source 1..28: mol_type = other DNA
agccgcacttcggccaagagcctgcagg

SEQ ID NO: 25221 - DNA, 28 bp, synthetic construct
  source 1..28: mol_type = other DNA
gcaggctcttggccgaagtgcggcttgg

SEQ ID NO: 25222 - DNA, 28 bp, synthetic construct
  source 1..28: mol_type = other DNA
caggctcttggccgaagtgcggcttggg

SEQ ID NO: 25223 - DNA, 28 bp, synthetic construct
  source 1..28: mol_type = other DNA
ctcttggccgaagtgcggcttgggacgg

SEQ ID NO: 25224 - DNA, 28 bp, synthetic construct
  source 1..28: mol_type = other DNA
tcttggccgaagtgcggcttgggacggg

SEQ ID NO: 25225 - DNA, 28 bp, synthetic construct
  source 1..28: mol_type = other DNA
cagcatcccgtcccaagccgcacttcgg

SEQ ID NO: 25226 - DNA, 28 bp, synthetic construct
  source 1..28: mol_type = other DNA
gcggcttgggacgggatgctgcgcgcgg

SEQ ID NO: 25227 - DNA, 28 bp, synthetic construct
  source 1..28: mol_type = other DNA
cggcttgggacgggatgctgcgcgcggg

SEQ ID NO: 25228 - DNA, 28 bp, synthetic construct
  source 1..28: mol_type = other DNA
tgggacgggatgctgcgcgcgggcctgg

SEQ ID NO: 25229 - DNA, 28 bp, synthetic construct
  source 1..28: mol_type = other DNA
gggatgctgcgcgcgggcctggtgaagg

SEQ ID NO: 25230 - DNA, 28 bp, synthetic construct
  source 1..28: mol_type = other DNA
ggatgctgcgcgcgggcctggtgaaggg

SEQ ID NO: 25231 - DNA, 28 bp, synthetic construct
  source 1..28: mol_type = other DNA
gcgcgcgggcctggtgaagggtcgtagg

SEQ ID NO: 25232 - DNA, 28 bp, synthetic construct
  source 1..28: mol_type = other DNA
cgggcctggtgaagggtcgtaggtccgg

SEQ ID NO: 25233 - DNA, 28 bp, synthetic construct
  source 1..28: mol_type = other DNA
gggcctggtgaagggtcgtaggtccggg

SEQ ID NO: 25234 - DNA, 28 bp, synthetic construct
  source 1..28: mol_type = other DNA
ctgcccggacctacgacccttcaccagg

SEQ ID NO: 25235 - DNA, 28 bp, synthetic construct
  source 1..28: mol_type = other DNA
ctggtgaagggtcgtaggtccgggcagg

SEQ ID NO: 25236 - DNA, 28 bp, synthetic construct
  source 1..28: mol_type = other DNA
gtgaagggtcgtaggtccgggcaggagg

SEQ ID NO: 25237 - DNA, 28 bp, synthetic construct
  source 1..28: mol_type = other DNA
gggtcgtaggtccgggcaggaggagagg

SEQ ID NO: 25238 - DNA, 28 bp, synthetic construct
  source 1..28: mol_type = other DNA
ggcacgcgctgcctctcctcctgcccgg

SEQ ID NO: 25239 - DNA, 28 bp, synthetic construct
  source 1..28: mol_type = other DNA
aggaggagaggcagcgcgtgcctttcgg

SEQ ID NO: 25240 - DNA, 28 bp, synthetic construct
  source 1..28: mol_type = other DNA
agaggcagcgcgtgcctttcggcgccgg

SEQ ID NO: 25241 - DNA, 28 bp, synthetic construct
  source 1..28: mol_type = other DNA
cagcgcgtgcctttcggcgccggcccgg

SEQ ID NO: 25242 - DNA, 28 bp, synthetic construct
  source 1..28: mol_type = other DNA
agcgcgtgcctttcggcgccggcccggg

SEQ ID NO: 25243 - DNA, 28 bp, synthetic construct
  source 1..28: mol_type = other DNA
cctcagctcccgggccggcgccgaaagg

SEQ ID NO: 25244 - DNA, 28 bp, synthetic construct
  source 1..28: mol_type = other DNA
acgagcaggtcctcagctcccgggccgg

SEQ ID NO: 25245 - DNA, 28 bp, synthetic construct
  source 1..28: mol_type = other DNA
tactacgagcaggtcctcagctcccggg

SEQ ID NO: 25246 - DNA, 28 bp, synthetic construct
  source 1..28: mol_type = other DNA
atactacgagcaggtcctcagctcccgg

SEQ ID NO: 25247 - DNA, 28 bp, synthetic construct
  source 1..28: mol_type = other DNA
ggagctgaggacctgctcgtagtatcgg

SEQ ID NO: 25248 - DNA, 28 bp, synthetic construct
  source 1..28: mol_type = other DNA
gagctgaggacctgctcgtagtatcggg

SEQ ID NO: 25249 - DNA, 28 bp, synthetic construct
  source 1..28: mol_type = other DNA
gggcgcacagcccgatactacgagcagg

SEQ ID NO: 25250 - DNA, 28 bp, synthetic construct
  source 1..28: mol_type = other DNA
cgtagtatcgggctgtgcgcccagctgg

SEQ ID NO: 25251 - DNA, 28 bp, synthetic construct
  source 1..28: mol_type = other DNA
gcgcccagctggaaagtctcgccgccgg

SEQ ID NO: 25252 - DNA, 28 bp, synthetic construct
  source 1..28: mol_type = other DNA
gagccggcggcgagactttccagctggg

SEQ ID NO: 25253 - DNA, 28 bp, synthetic construct
  source 1..28: mol_type = other DNA
ggagccggcggcgagactttccagctgg

SEQ ID NO: 25254 - DNA, 28 bp, synthetic construct
  source 1..28: mol_type = other DNA
agctggaaagtctcgccgccggctccgg

SEQ ID NO: 25255 - DNA, 28 bp, synthetic construct
  source 1..28: mol_type = other DNA
gctactctgagggcgccggagccggcgg

SEQ ID NO: 25256 - DNA, 28 bp, synthetic construct
  source 1..28: mol_type = other DNA
gccggctccggcgccctcagagtagcgg

SEQ ID NO: 25257 - DNA, 28 bp, synthetic construct
  source 1..28: mol_type = other DNA
gccgctactctgagggcgccggagccgg

SEQ ID NO: 25258 - DNA, 28 bp, synthetic construct
  source 1..28: mol_type = other DNA
tgcgcggccgctactctgagggcgccgg

SEQ ID NO: 25259 - DNA, 28 bp, synthetic construct
  source 1..28: mol_type = other DNA
tcacactgcgcggccgctactctgaggg

SEQ ID NO: 25260 - DNA, 28 bp, synthetic construct
  source 1..28: mol_type = other DNA
ctcacactgcgcggccgctactctgagg

SEQ ID NO: 25261 - DNA, 28 bp, synthetic construct
  source 1..28: mol_type = other DNA
ctcagagtagcggccgcgcagtgtgagg

SEQ ID NO: 25262 - DNA, 28 bp, synthetic construct
  source 1..28: mol_type = other DNA
tcagagtagcggccgcgcagtgtgaggg

SEQ ID NO: 25263 - DNA, 28 bp, synthetic construct
  source 1..28: mol_type = other DNA
agacacgaaacaccctcacactgcgcgg

SEQ ID NO: 25264 - DNA, 28 bp, synthetic construct
  source 1..28: mol_type = other DNA
cgcagtgtgagggtgtttcgtgtcttgg

SEQ ID NO: 25265 - DNA, 28 bp, synthetic construct
  source 1..28: mol_type = other DNA
gagggtgtttcgtgtcttggttttttgg

SEQ ID NO: 25266 - DNA, 28 bp, synthetic construct
  source 1..28: mol_type = other DNA
agggtgtttcgtgtcttggttttttggg

SEQ ID NO: 25267 - DNA, 28 bp, synthetic construct
  source 1..28: mol_type = other DNA
gggtgtttcgtgtcttggttttttgggg

SEQ ID NO: 25268 - DNA, 28 bp, synthetic construct
  source 1..28: mol_type = other DNA
tcgtgtcttggttttttggggcgcgtgg

SEQ ID NO: 25269 - DNA, 28 bp, synthetic construct
  source 1..28: mol_type = other DNA
cgtgtcttggttttttggggcgcgtggg

SEQ ID NO: 25270 - DNA, 28 bp, synthetic construct
  source 1..28: mol_type = other DNA
ttttttggggcgcgtgggcctgttgcgg

SEQ ID NO: 25271 - DNA, 28 bp, synthetic construct
  source 1..28: mol_type = other DNA
tttggggcgcgtgggcctgttgcggagg

SEQ ID NO: 25272 - DNA, 28 bp, synthetic construct
  source 1..28: mol_type = other DNA
gcgtgggcctgttgcggaggatttgcgg

SEQ ID NO: 25273 - DNA, 28 bp, synthetic construct
  source 1..28: mol_type = other DNA
cgcagttccgcaaatcctccgcaacagg

SEQ ID NO: 25274 - DNA, 28 bp, synthetic construct
  source 1..28: mol_type = other DNA
ctgttgcggaggatttgcggaactgcgg

SEQ ID NO: 25275 - DNA, 28 bp, synthetic construct
  source 1..28: mol_type = other DNA
ttgcggaggatttgcggaactgcggtgg

SEQ ID NO: 25276 - DNA, 28 bp, synthetic construct
  source 1..28: mol_type = other DNA
cggtggtgatttaactgacgagacacgg

SEQ ID NO: 25277 - DNA, 28 bp, synthetic construct
  source 1..28: mol_type = other DNA
acacggcttttccttttactcattcagg

SEQ ID NO: 25278 - DNA, 28 bp, synthetic construct
  source 1..28: mol_type = other DNA
cttttccttttactcattcaggccaagg

SEQ ID NO: 25279 - DNA, 28 bp, synthetic construct
  source 1..28: mol_type = other DNA
cgaaaccttggcctgaatgagtaaaagg

SEQ ID NO: 25280 - DNA, 28 bp, synthetic construct
  source 1..28: mol_type = other DNA
cttttactcattcaggccaaggtttcgg

SEQ ID NO: 25281 - DNA, 28 bp, synthetic construct
  source 1..28: mol_type = other DNA
ttttactcattcaggccaaggtttcggg

SEQ ID NO: 25282 - DNA, 28 bp, synthetic construct
  source 1..28: mol_type = other DNA
tttactcattcaggccaaggtttcgggg

SEQ ID NO: 25283 - DNA, 28 bp, synthetic construct
  source 1..28: mol_type = other DNA
gaacgcagcagtggccccgaaaccttgg

SEQ ID NO: 25284 - DNA, 28 bp, synthetic construct
  source 1..28: mol_type = other DNA
acgcttgagaaagcgaacgcagcagtgg

SEQ ID NO: 25285 - DNA, 28 bp, synthetic construct
  source 1..28: mol_type = other DNA
ctgcgttcgctttctcaagcgtacctgg

SEQ ID NO: 25286 - DNA, 28 bp, synthetic construct
  source 1..28: mol_type = other DNA
tgcgttcgctttctcaagcgtacctggg

SEQ ID NO: 25287 - DNA, 28 bp, synthetic construct
  source 1..28: mol_type = other DNA
gcgttcgctttctcaagcgtacctgggg

SEQ ID NO: 25288 - DNA, 28 bp, synthetic construct
  source 1..28: mol_type = other DNA
tacctggggcccctgcttgctctgcagg

SEQ ID NO: 25289 - DNA, 28 bp, synthetic construct
  source 1..28: mol_type = other DNA
ctcctgcagagcaagcaggggccccagg

SEQ ID NO: 25290 - DNA, 28 bp, synthetic construct
  source 1..28: mol_type = other DNA
cgcaggactcctgcagagcaagcagggg

SEQ ID NO: 25291 - DNA, 28 bp, synthetic construct
  source 1..28: mol_type = other DNA
ccgcaggactcctgcagagcaagcaggg

SEQ ID NO: 25292 - DNA, 28 bp, synthetic construct
  source 1..28: mol_type = other DNA
gccgcaggactcctgcagagcaagcagg

SEQ ID NO: 25293 - DNA, 28 bp, synthetic construct
  source 1..28: mol_type = other DNA
gaatcgtgcggatggcacaggccgcagg

SEQ ID NO: 25294 - DNA, 28 bp, synthetic construct
  source 1..28: mol_type = other DNA
ggcctgtgccatccgcacgattccctgg

SEQ ID NO: 25295 - DNA, 28 bp, synthetic construct
  source 1..28: mol_type = other DNA
tgccagggaatcgtgcggatggcacagg

SEQ ID NO: 25296 - DNA, 28 bp, synthetic construct
  source 1..28: mol_type = other DNA
tctcgctgccagggaatcgtgcggatgg

SEQ ID NO: 25297 - DNA, 28 bp, synthetic construct
  source 1..28: mol_type = other DNA
gatttctcgctgccagggaatcgtgcgg

SEQ ID NO: 25298 - DNA, 28 bp, synthetic construct
  source 1..28: mol_type = other DNA
acgattccctggcagcgagaaatctagg

SEQ ID NO: 25299 - DNA, 28 bp, synthetic construct
  source 1..28: mol_type = other DNA
ggaggacctagatttctcgctgccaggg

SEQ ID NO: 25300 - DNA, 28 bp, synthetic construct
  source 1..28: mol_type = other DNA
gggaggacctagatttctcgctgccagg

SEQ ID NO: 25301 - DNA, 28 bp, synthetic construct
  source 1..28: mol_type = other DNA
aaatctaggtcctcccctgaccacctgg

SEQ ID NO: 25302 - DNA, 28 bp, synthetic construct
  source 1..28: mol_type = other DNA
cctgcgcggtccaggtggtcaggggagg

SEQ ID NO: 25303 - DNA, 28 bp, synthetic construct
  source 1..28: mol_type = other DNA
ctcccctgaccacctggaccgcgcaggg

SEQ ID NO: 25304 - DNA, 28 bp, synthetic construct
  source 1..28: mol_type = other DNA
tcccctgaccacctggaccgcgcagggg

SEQ ID NO: 25305 - DNA, 28 bp, synthetic construct
  source 1..28: mol_type = other DNA
tcccctgcgcggtccaggtggtcagggg

SEQ ID NO: 25306 - DNA, 28 bp, synthetic construct
  source 1..28: mol_type = other DNA
gtcccctgcgcggtccaggtggtcaggg

SEQ ID NO: 25307 - DNA, 28 bp, synthetic construct
  source 1..28: mol_type = other DNA
agtcccctgcgcggtccaggtggtcagg

SEQ ID NO: 25308 - DNA, 28 bp, synthetic construct
  source 1..28: mol_type = other DNA
cgactagtcccctgcgcggtccaggtgg

SEQ ID NO: 25309 - DNA, 28 bp, synthetic construct
  source 1..28: mol_type = other DNA
ccgcgactagtcccctgcgcggtccagg

SEQ ID NO: 25310 - DNA, 28 bp, synthetic construct
  source 1..28: mol_type = other DNA
gaccgcgcaggggactagtcgcggccgg

SEQ ID NO: 25311 - DNA, 28 bp, synthetic construct
  source 1..28: mol_type = other DNA
tgccggccgcgactagtcccctgcgcgg

SEQ ID NO: 25312 - DNA, 28 bp, synthetic construct
  source 1..28: mol_type = other DNA
ctagtcgcggccggcagaacctgctcgg

SEQ ID NO: 25313 - DNA, 28 bp, synthetic construct
  source 1..28: mol_type = other DNA
cggccggcagaacctgctcggtccctgg

SEQ ID NO: 25314 - DNA, 28 bp, synthetic construct
  source 1..28: mol_type = other DNA
ggccggcagaacctgctcggtccctggg

SEQ ID NO: 25315 - DNA, 28 bp, synthetic construct
  source 1..28: mol_type = other DNA
ggcccagggaccgagcaggttctgccgg

SEQ ID NO: 25316 - DNA, 28 bp, synthetic construct
  source 1..28: mol_type = other DNA
ggcagaacctgctcggtccctgggccgg

SEQ ID NO: 25317 - DNA, 28 bp, synthetic construct
  source 1..28: mol_type = other DNA
gcagaacctgctcggtccctgggccggg

SEQ ID NO: 25318 - DNA, 28 bp, synthetic construct
  source 1..28: mol_type = other DNA
agatagcccggcccagggaccgagcagg

SEQ ID NO: 25319 - DNA, 28 bp, synthetic construct
  source 1..28: mol_type = other DNA
cggtccctgggccgggctatcttagcgg

SEQ ID NO: 25320 - DNA, 28 bp, synthetic construct
  source 1..28: mol_type = other DNA
tgagccgctaagatagcccggcccaggg

SEQ ID NO: 25321 - DNA, 28 bp, synthetic construct
  source 1..28: mol_type = other DNA
gtgagccgctaagatagcccggcccagg

SEQ ID NO: 25322 - DNA, 28 bp, synthetic construct
  source 1..28: mol_type = other DNA
gcatgcgtgagccgctaagatagcccgg

SEQ ID NO: 25323 - DNA, 28 bp, synthetic construct
  source 1..28: mol_type = other DNA
cacgcatgcccgagcacacccgacccgg

SEQ ID NO: 25324 - DNA, 28 bp, synthetic construct
  source 1..28: mol_type = other DNA
gcccgagcacacccgacccggttcgcgg

SEQ ID NO: 25325 - DNA, 28 bp, synthetic construct
  source 1..28: mol_type = other DNA
accgcgaaccgggtcgggtgtgctcggg

SEQ ID NO: 25326 - DNA, 28 bp, synthetic construct
  source 1..28: mol_type = other DNA
caccgcgaaccgggtcgggtgtgctcgg

SEQ ID NO: 25327 - DNA, 28 bp, synthetic construct
  source 1..28: mol_type = other DNA
gcacacccgacccggttcgcggtgcagg

SEQ ID NO: 25328 - DNA, 28 bp, synthetic construct
  source 1..28: mol_type = other DNA
acccgacccggttcgcggtgcaggctgg

SEQ ID NO: 25329 - DNA, 28 bp, synthetic construct
  source 1..28: mol_type = other DNA
gccagcctgcaccgcgaaccgggtcggg

SEQ ID NO: 25330 - DNA, 28 bp, synthetic construct
  source 1..28: mol_type = other DNA
cgccagcctgcaccgcgaaccgggtcgg

SEQ ID NO: 25331 - DNA, 28 bp, synthetic construct
  source 1..28: mol_type = other DNA
cgacccggttcgcggtgcaggctggcgg

SEQ ID NO: 25332 - DNA, 28 bp, synthetic construct
  source 1..28: mol_type = other DNA
gcgccgccagcctgcaccgcgaaccggg

SEQ ID NO: 25333 - DNA, 28 bp, synthetic construct
  source 1..28: mol_type = other DNA
ggcgccgccagcctgcaccgcgaaccgg

SEQ ID NO: 25334 - DNA, 28 bp, synthetic construct
  source 1..28: mol_type = other DNA
tgcaggctggcggcgccgtgccctctgg

SEQ ID NO: 25335 - DNA, 28 bp, synthetic construct
  source 1..28: mol_type = other DNA
gcaggctggcggcgccgtgccctctggg

SEQ ID NO: 25336 - DNA, 28 bp, synthetic construct
  source 1..28: mol_type = other DNA
ctggggcaacaggtcccagagggcacgg

SEQ ID NO: 25337 - DNA, 28 bp, synthetic construct
  source 1..28: mol_type = other DNA
cgtgccctctgggacctgttgccccagg

SEQ ID NO: 25338 - DNA, 28 bp, synthetic construct
  source 1..28: mol_type = other DNA
gtgccctctgggacctgttgccccaggg

SEQ ID NO: 25339 - DNA, 28 bp, synthetic construct
  source 1..28: mol_type = other DNA
caaccctggggcaacaggtcccagaggg

SEQ ID NO: 25340 - DNA, 28 bp, synthetic construct
  source 1..28: mol_type = other DNA
cctctgggacctgttgccccagggttgg

SEQ ID NO: 25341 - DNA, 28 bp, synthetic construct
  source 1..28: mol_type = other DNA
cctgttgccccagggttggcgctgctgg

SEQ ID NO: 25342 - DNA, 28 bp, synthetic construct
  source 1..28: mol_type = other DNA
gttgccccagggttggcgctgctggtgg

SEQ ID NO: 25343 - DNA, 28 bp, synthetic construct
  source 1..28: mol_type = other DNA
gccccagggttggcgctgctggtggagg

SEQ ID NO: 25344 - DNA, 28 bp, synthetic construct
  source 1..28: mol_type = other DNA
ccctccaccagcagcgccaaccctgggg

SEQ ID NO: 25345 - DNA, 28 bp, synthetic construct
  source 1..28: mol_type = other DNA
gccctccaccagcagcgccaaccctggg

SEQ ID NO: 25346 - DNA, 28 bp, synthetic construct
  source 1..28: mol_type = other DNA
ggccctccaccagcagcgccaaccctgg

SEQ ID NO: 25347 - DNA, 28 bp, synthetic construct
  source 1..28: mol_type = other DNA
ttggcgctgctggtggagggcccgacgg

SEQ ID NO: 25348 - DNA, 28 bp, synthetic construct
  source 1..28: mol_type = other DNA
gctggtggagggcccgacggacgccagg

SEQ ID NO: 25349 - DNA, 28 bp, synthetic construct
  source 1..28: mol_type = other DNA
ctggtggagggcccgacggacgccaggg

SEQ ID NO: 25350 - DNA, 28 bp, synthetic construct
  source 1..28: mol_type = other DNA
gtggagggcccgacggacgccagggcgg

SEQ ID NO: 25351 - DNA, 28 bp, synthetic construct
  source 1..28: mol_type = other DNA
gagggcccgacggacgccagggcggagg

SEQ ID NO: 25352 - DNA, 28 bp, synthetic construct
  source 1..28: mol_type = other DNA
agggcccgacggacgccagggcggaggg

SEQ ID NO: 25353 - DNA, 28 bp, synthetic construct
  source 1..28: mol_type = other DNA
cacaccctccgccctggcgtccgtcggg

SEQ ID NO: 25354 - DNA, 28 bp, synthetic construct
  source 1..28: mol_type = other DNA
tcacaccctccgccctggcgtccgtcgg

SEQ ID NO: 25355 - DNA, 28 bp, synthetic construct
  source 1..28: mol_type = other DNA
tcgagtaaattcacaccctccgccctgg

SEQ ID NO: 25356 - DNA, 28 bp, synthetic construct
  source 1..28: mol_type = other DNA
gggcggagggtgtgaatttactcgatgg

SEQ ID NO: 25357 - DNA, 28 bp, synthetic construct
  source 1..28: mol_type = other DNA
agggtgtgaatttactcgatggtcgcgg

SEQ ID NO: 25358 - DNA, 28 bp, synthetic construct
  source 1..28: mol_type = other DNA
cgatggtcgcggacgtgcgcgtccgcgg

SEQ ID NO: 25359 - DNA, 28 bp, synthetic construct
  source 1..28: mol_type = other DNA
gtcgcggacgtgcgcgtccgcggccagg

SEQ ID NO: 25360 - DNA, 28 bp, synthetic construct
  source 1..28: mol_type = other DNA
tcgcggacgtgcgcgtccgcggccaggg

SEQ ID NO: 25361 - DNA, 28 bp, synthetic construct
  source 1..28: mol_type = other DNA
cgcggacgtgcgcgtccgcggccagggg

SEQ ID NO: 25362 - DNA, 28 bp, synthetic construct
  source 1..28: mol_type = other DNA
ggacgtgcgcgtccgcggccaggggtgg

SEQ ID NO: 25363 - DNA, 28 bp, synthetic construct
  source 1..28: mol_type = other DNA
gcgtccgcggccaggggtggctcttcgg

SEQ ID NO: 25364 - DNA, 28 bp, synthetic construct
  source 1..28: mol_type = other DNA
aaagccgaagagccacccctggccgcgg

SEQ ID NO: 25365 - DNA, 28 bp, synthetic construct
  source 1..28: mol_type = other DNA
cgagtcaaagccgaagagccacccctgg

SEQ ID NO: 25366 - DNA, 28 bp, synthetic construct
  source 1..28: mol_type = other DNA
gctcttcggctttgactcgtgtctgcgg

SEQ ID NO: 25367 - DNA, 28 bp, synthetic construct
  source 1..28: mol_type = other DNA
ctttgactcgtgtctgcggcgcaccagg

SEQ ID NO: 25368 - DNA, 28 bp, synthetic construct
  source 1..28: mol_type = other DNA
gtgtctgcggcgcaccaggagagagagg

SEQ ID NO: 25369 - DNA, 28 bp, synthetic construct
  source 1..28: mol_type = other DNA
cgcaccaggagagagaggaagttgttgg

SEQ ID NO: 25370 - DNA, 28 bp, synthetic construct
  source 1..28: mol_type = other DNA
accaggagagagaggaagttgttggagg

SEQ ID NO: 25371 - DNA, 28 bp, synthetic construct
  source 1..28: mol_type = other DNA
tcctccaacaacttcctctctctcctgg

SEQ ID NO: 25372 - DNA, 28 bp, synthetic construct
  source 1..28: mol_type = other DNA
ttggaggagaatagttgccacagccagg

SEQ ID NO: 25373 - DNA, 28 bp, synthetic construct
  source 1..28: mol_type = other DNA
tggaggagaatagttgccacagccaggg

SEQ ID NO: 25374 - DNA, 28 bp, synthetic construct
  source 1..28: mol_type = other DNA
aggagaatagttgccacagccagggcgg

SEQ ID NO: 25375 - DNA, 28 bp, synthetic construct
  source 1..28: mol_type = other DNA
atagttgccacagccagggcggtgacgg

SEQ ID NO: 25376 - DNA, 28 bp, synthetic construct
  source 1..28: mol_type = other DNA
ctaacggccgtcaccgccctggctgtgg

SEQ ID NO: 25377 - DNA, 28 bp, synthetic construct
  source 1..28: mol_type = other DNA
cacagccagggcggtgacggccgttagg

SEQ ID NO: 25378 - DNA, 28 bp, synthetic construct
  source 1..28: mol_type = other DNA
acagccagggcggtgacggccgttaggg

SEQ ID NO: 25379 - DNA, 28 bp, synthetic construct
  source 1..28: mol_type = other DNA
cagaccctaacggccgtcaccgccctgg

SEQ ID NO: 25380 - DNA, 28 bp, synthetic construct
  source 1..28: mol_type = other DNA
gacggccgttagggtctgcccccgacgg

SEQ ID NO: 25381 - DNA, 28 bp, synthetic construct
  source 1..28: mol_type = other DNA
acggccgttagggtctgcccccgacggg

SEQ ID NO: 25382 - DNA, 28 bp, synthetic construct
  source 1..28: mol_type = other DNA
ttggcccgtcgggggcagaccctaacgg

SEQ ID NO: 25383 - DNA, 28 bp, synthetic construct
  source 1..28: mol_type = other DNA
ggtctgcccccgacgggccaaaacaagg

SEQ ID NO: 25384 - DNA, 28 bp, synthetic construct
  source 1..28: mol_type = other DNA
acttgtccttgttttggcccgtcggggg

SEQ ID NO: 25385 - DNA, 28 bp, synthetic construct
  source 1..28: mol_type = other DNA
cacttgtccttgttttggcccgtcgggg

SEQ ID NO: 25386 - DNA, 28 bp, synthetic construct
  source 1..28: mol_type = other DNA
ccacttgtccttgttttggcccgtcggg

SEQ ID NO: 25387 - DNA, 28 bp, synthetic construct
  source 1..28: mol_type = other DNA
gccacttgtccttgttttggcccgtcgg

SEQ ID NO: 25388 - DNA, 28 bp, synthetic construct
  source 1..28: mol_type = other DNA
cgggccaaaacaaggacaagtggcgagg

SEQ ID NO: 25389 - DNA, 28 bp, synthetic construct
  source 1..28: mol_type = other DNA
cagtcctcgccacttgtccttgttttgg

SEQ ID NO: 25390 - DNA, 28 bp, synthetic construct
  source 1..28: mol_type = other DNA
caaaacaaggacaagtggcgaggactgg

SEQ ID NO: 25391 - DNA, 28 bp, synthetic construct
  source 1..28: mol_type = other DNA
aaaacaaggacaagtggcgaggactggg

SEQ ID NO: 25392 - DNA, 28 bp, synthetic construct
  source 1..28: mol_type = other DNA
aaggacaagtggcgaggactgggcctgg

SEQ ID NO: 25393 - DNA, 28 bp, synthetic construct
  source 1..28: mol_type = other DNA
aggacaagtggcgaggactgggcctggg

SEQ ID NO: 25394 - DNA, 28 bp, synthetic construct
  source 1..28: mol_type = other DNA
ggacaagtggcgaggactgggcctgggg

SEQ ID NO: 25395 - DNA, 28 bp, synthetic construct
  source 1..28: mol_type = other DNA
aagtggcgaggactgggcctggggatgg

SEQ ID NO: 25396 - DNA, 28 bp, synthetic construct
  source 1..28: mol_type = other DNA
aggactgggcctggggatggccctgcgg

SEQ ID NO: 25397 - DNA, 28 bp, synthetic construct
  source 1..28: mol_type = other DNA
ggactgggcctggggatggccctgcggg

SEQ ID NO: 25398 - DNA, 28 bp, synthetic construct
  source 1..28: mol_type = other DNA
gggcctggggatggccctgcgggtccgg

SEQ ID NO: 25399 - DNA, 28 bp, synthetic construct
  source 1..28: mol_type = other DNA
ggcctggggatggccctgcgggtccggg

SEQ ID NO: 25400 - DNA, 28 bp, synthetic construct
  source 1..28: mol_type = other DNA
cgcccggacccgcagggccatccccagg

SEQ ID NO: 25401 - DNA, 28 bp, synthetic construct
  source 1..28: mol_type = other DNA
ggggatggccctgcgggtccgggcgcgg

SEQ ID NO: 25402 - DNA, 28 bp, synthetic construct
  source 1..28: mol_type = other DNA
gacttgcgccgcgcccggacccgcaggg

SEQ ID NO: 25403 - DNA, 28 bp, synthetic construct
  source 1..28: mol_type = other DNA
ggacttgcgccgcgcccggacccgcagg

SEQ ID NO: 25404 - DNA, 28 bp, synthetic construct
  source 1..28: mol_type = other DNA
gacaaagcaggacttgcgccgcgcccgg

SEQ ID NO: 25405 - DNA, 28 bp, synthetic construct
  source 1..28: mol_type = other DNA
gcggcgcaagtcctgctttgtctccagg

SEQ ID NO: 25406 - DNA, 28 bp, synthetic construct
  source 1..28: mol_type = other DNA
aagtcctgctttgtctccaggtgactgg

SEQ ID NO: 25407 - DNA, 28 bp, synthetic construct
  source 1..28: mol_type = other DNA
acagccagtcacctggagacaaagcagg

SEQ ID NO: 25408 - DNA, 28 bp, synthetic construct
  source 1..28: mol_type = other DNA
tttgtctccaggtgactggctgtccagg

SEQ ID NO: 25409 - DNA, 28 bp, synthetic construct
  source 1..28: mol_type = other DNA
tctccaggtgactggctgtccaggacgg

SEQ ID NO: 25410 - DNA, 28 bp, synthetic construct
  source 1..28: mol_type = other DNA
ccaggtgactggctgtccaggacggcgg

SEQ ID NO: 25411 - DNA, 28 bp, synthetic construct
  source 1..28: mol_type = other DNA
caggtgactggctgtccaggacggcggg

SEQ ID NO: 25412 - DNA, 28 bp, synthetic construct
  source 1..28: mol_type = other DNA
ctgtccaggacggcgggagctgctaagg

SEQ ID NO: 25413 - DNA, 28 bp, synthetic construct
  source 1..28: mol_type = other DNA
caagccttagcagctcccgccgtcctgg

SEQ ID NO: 25414 - DNA, 28 bp, synthetic construct
  source 1..28: mol_type = other DNA
ggcgggagctgctaaggcttgtgtccgg

SEQ ID NO: 25415 - DNA, 28 bp, synthetic construct
  source 1..28: mol_type = other DNA
ggagctgctaaggcttgtgtccggaagg

SEQ ID NO: 25416 - DNA, 28 bp, synthetic construct
  source 1..28: mol_type = other DNA
taaggcttgtgtccggaaggagcacagg

SEQ ID NO: 25417 - DNA, 28 bp, synthetic construct
  source 1..28: mol_type = other DNA
aaggcttgtgtccggaaggagcacaggg

SEQ ID NO: 25418 - DNA, 28 bp, synthetic construct
  source 1..28: mol_type = other DNA
cttgtgtccggaaggagcacagggatgg

SEQ ID NO: 25419 - DNA, 28 bp, synthetic construct
  source 1..28: mol_type = other DNA
ttgtgtccggaaggagcacagggatggg

SEQ ID NO: 25420 - DNA, 28 bp, synthetic construct
  source 1..28: mol_type = other DNA
gtccggaaggagcacagggatgggcagg

SEQ ID NO: 25421 - DNA, 28 bp, synthetic construct
  source 1..28: mol_type = other DNA
tccggaaggagcacagggatgggcaggg

SEQ ID NO: 25422 - DNA, 28 bp, synthetic construct
  source 1..28: mol_type = other DNA
accctgcccatccctgtgctccttccgg

SEQ ID NO: 25423 - DNA, 28 bp, synthetic construct
  source 1..28: mol_type = other DNA
ggaaggagcacagggatgggcagggtgg

SEQ ID NO: 25424 - DNA, 28 bp, synthetic construct
  source 1..28: mol_type = other DNA
ggagcacagggatgggcagggtggccgg

SEQ ID NO: 25425 - DNA, 28 bp, synthetic construct
  source 1..28: mol_type = other DNA
gagcacagggatgggcagggtggccggg

SEQ ID NO: 25426 - DNA, 28 bp, synthetic construct
  source 1..28: mol_type = other DNA
ggatgggcagggtggccgggccagccgg

SEQ ID NO: 25427 - DNA, 28 bp, synthetic construct
  source 1..28: mol_type = other DNA
cggaggatttgagggccggctggcccgg

SEQ ID NO: 25428 - DNA, 28 bp, synthetic construct
  source 1..28: mol_type = other DNA
ttcgtcggaggatttgagggccggctgg

SEQ ID NO: 25429 - DNA, 28 bp, synthetic construct
  source 1..28: mol_type = other DNA
ccggccctcaaatcctccgacgaagcgg

SEQ ID NO: 25430 - DNA, 28 bp, synthetic construct
  source 1..28: mol_type = other DNA
gctgccgcttcgtcggaggatttgaggg

SEQ ID NO: 25431 - DNA, 28 bp, synthetic construct
  source 1..28: mol_type = other DNA
ggctgccgcttcgtcggaggatttgagg

SEQ ID NO: 25432 - DNA, 28 bp, synthetic construct
  source 1..28: mol_type = other DNA
gtcgtggcggctgccgcttcgtcggagg

SEQ ID NO: 25433 - DNA, 28 bp, synthetic construct
  source 1..28: mol_type = other DNA
gtggtcgtggcggctgccgcttcgtcgg

SEQ ID NO: 25434 - DNA, 28 bp, synthetic construct
  source 1..28: mol_type = other DNA
gacgaagcggcagccgccacgaccacgg

SEQ ID NO: 25435 - DNA, 28 bp, synthetic construct
  source 1..28: mol_type = other DNA
agcgctgctctggccgtggtcgtggcgg

SEQ ID NO: 25436 - DNA, 28 bp, synthetic construct
  source 1..28: mol_type = other DNA
ccacgaccacggccagagcagcgctcgg

SEQ ID NO: 25437 - DNA, 28 bp, synthetic construct
  source 1..28: mol_type = other DNA
cgaccacggccagagcagcgctcggagg

SEQ ID NO: 25438 - DNA, 28 bp, synthetic construct
  source 1..28: mol_type = other DNA
tcgcctccgagcgctgctctggccgtgg

SEQ ID NO: 25439 - DNA, 28 bp, synthetic construct
  source 1..28: mol_type = other DNA
acaaactcgcctccgagcgctgctctgg

SEQ ID NO: 25440 - DNA, 28 bp, synthetic construct
  source 1..28: mol_type = other DNA
agtttgtcaacaatcgcctcgcctttgg

SEQ ID NO: 25441 - DNA, 28 bp, synthetic construct
  source 1..28: mol_type = other DNA
ttgtcaacaatcgcctcgcctttggcgg

SEQ ID NO: 25442 - DNA, 28 bp, synthetic construct
  source 1..28: mol_type = other DNA
cctacgggtcaggccgccaaaggcgagg

SEQ ID NO: 25443 - DNA, 28 bp, synthetic construct
  source 1..28: mol_type = other DNA
cggcgcctacgggtcaggccgccaaagg

SEQ ID NO: 25444 - DNA, 28 bp, synthetic construct
  source 1..28: mol_type = other DNA
gcggtgggggcggcgcctacgggtcagg

SEQ ID NO: 25445 - DNA, 28 bp, synthetic construct
  source 1..28: mol_type = other DNA
tgacccgtaggcgccgcccccaccgcgg

SEQ ID NO: 25446 - DNA, 28 bp, synthetic construct
  source 1..28: mol_type = other DNA
cagccgcggtgggggcggcgcctacggg

SEQ ID NO: 25447 - DNA, 28 bp, synthetic construct
  source 1..28: mol_type = other DNA
gcagccgcggtgggggcggcgcctacgg

SEQ ID NO: 25448 - DNA, 28 bp, synthetic construct
  source 1..28: mol_type = other DNA
cgccgcccccaccgcggctgccgattgg

SEQ ID NO: 25449 - DNA, 28 bp, synthetic construct
  source 1..28: mol_type = other DNA
agccaatcggcagccgcggtgggggcgg

SEQ ID NO: 25450 - DNA, 28 bp, synthetic construct
  source 1..28: mol_type = other DNA
cgcagccaatcggcagccgcggtggggg

SEQ ID NO: 25451 - DNA, 28 bp, synthetic construct
  source 1..28: mol_type = other DNA
ccccaccgcggctgccgattggctgcgg

SEQ ID NO: 25452 - DNA, 28 bp, synthetic construct
  source 1..28: mol_type = other DNA
gccgcagccaatcggcagccgcggtggg

SEQ ID NO: 25453 - DNA, 28 bp, synthetic construct
  source 1..28: mol_type = other DNA
cgccgcagccaatcggcagccgcggtgg

SEQ ID NO: 25454 - DNA, 28 bp, synthetic construct
  source 1..28: mol_type = other DNA
ccgcggctgccgattggctgcggcgcgg

SEQ ID NO: 25455 - DNA, 28 bp, synthetic construct
  source 1..28: mol_type = other DNA
gcggtcgctccgcgccgcagccaatcgg

SEQ ID NO: 25456 - DNA, 28 bp, synthetic construct
  source 1..28: mol_type = other DNA
ggctgcggcgcggagcgaccgcgcgcgg

SEQ ID NO: 25457 - DNA, 28 bp, synthetic construct
  source 1..28: mol_type = other DNA
gcggagcgaccgcgcgcggaccaattgg

SEQ ID NO: 25458 - DNA, 28 bp, synthetic construct
  source 1..28: mol_type = other DNA
cggagcgaccgcgcgcggaccaattggg

SEQ ID NO: 25459 - DNA, 28 bp, synthetic construct
  source 1..28: mol_type = other DNA
accgcgcgcggaccaattgggaacgcgg

SEQ ID NO: 25460 - DNA, 28 bp, synthetic construct
  source 1..28: mol_type = other DNA
ccgcgcgcggaccaattgggaacgcggg

SEQ ID NO: 25461 - DNA, 28 bp, synthetic construct
  source 1..28: mol_type = other DNA
cggaccaattgggaacgcgggcacccgg

SEQ ID NO: 25462 - DNA, 28 bp, synthetic construct
  source 1..28: mol_type = other DNA
ggcgccgggtgcccgcgttcccaattgg

SEQ ID NO: 25463 - DNA, 28 bp, synthetic construct
  source 1..28: mol_type = other DNA
tgggaacgcgggcacccggcgccagcgg

SEQ ID NO: 25464 - DNA, 28 bp, synthetic construct
  source 1..28: mol_type = other DNA
acgcgggcacccggcgccagcggcgcgg

SEQ ID NO: 25465 - DNA, 28 bp, synthetic construct
  source 1..28: mol_type = other DNA
cgcgggcacccggcgccagcggcgcggg

SEQ ID NO: 25466 - DNA, 28 bp, synthetic construct
  source 1..28: mol_type = other DNA
gcgggcacccggcgccagcggcgcgggg

SEQ ID NO: 25467 - DNA, 28 bp, synthetic construct
  source 1..28: mol_type = other DNA
ggcacccggcgccagcggcgcggggagg

SEQ ID NO: 25468 - DNA, 28 bp, synthetic construct
  source 1..28: mol_type = other DNA
ccgacctccccgcgccgctggcgccggg

SEQ ID NO: 25469 - DNA, 28 bp, synthetic construct
  source 1..28: mol_type = other DNA
gccgacctccccgcgccgctggcgccgg

SEQ ID NO: 25470 - DNA, 28 bp, synthetic construct
  source 1..28: mol_type = other DNA
ggcgccagcggcgcggggaggtcggcgg

SEQ ID NO: 25471 - DNA, 28 bp, synthetic construct
  source 1..28: mol_type = other DNA
ggcaccgccgacctccccgcgccgctgg

SEQ ID NO: 25472 - DNA, 28 bp, synthetic construct
  source 1..28: mol_type = other DNA
agcggcgcggggaggtcggcggtgccgg

SEQ ID NO: 25473 - DNA, 28 bp, synthetic construct
  source 1..28: mol_type = other DNA
ggcgcggggaggtcggcggtgccggcgg

SEQ ID NO: 25474 - DNA, 28 bp, synthetic construct
  source 1..28: mol_type = other DNA
gcggggaggtcggcggtgccggcggcgg

SEQ ID NO: 25475 - DNA, 28 bp, synthetic construct
  source 1..28: mol_type = other DNA
gggaggtcggcggtgccggcggcggcgg

SEQ ID NO: 25476 - DNA, 28 bp, synthetic construct
  source 1..28: mol_type = other DNA
ggaggtcggcggtgccggcggcggcggg

SEQ ID NO: 25477 - DNA, 28 bp, synthetic construct
  source 1..28: mol_type = other DNA
cctcgcgctctgcgcccgccgccgccgg

SEQ ID NO: 25478 - DNA, 28 bp, synthetic construct
  source 1..28: mol_type = other DNA
cggcggcggcgggcgcagagcgcgaggg

SEQ ID NO: 25479 - DNA, 28 bp, synthetic construct
  source 1..28: mol_type = other DNA
ggcggcggcgggcgcagagcgcgagggg

SEQ ID NO: 25480 - DNA, 28 bp, synthetic construct
  source 1..28: mol_type = other DNA
ggcggcgggcgcagagcgcgaggggagg

SEQ ID NO: 25481 - DNA, 28 bp, synthetic construct
  source 1..28: mol_type = other DNA
cgggcgcagagcgcgaggggaggagcgg

SEQ ID NO: 25482 - DNA, 28 bp, synthetic construct
  source 1..28: mol_type = other DNA
gggcgcagagcgcgaggggaggagcggg

SEQ ID NO: 25483 - DNA, 28 bp, synthetic construct
  source 1..28: mol_type = other DNA
cgcagagcgcgaggggaggagcgggagg

SEQ ID NO: 25484 - DNA, 28 bp, synthetic construct
  source 1..28: mol_type = other DNA
agagcgcgaggggaggagcgggaggagg

SEQ ID NO: 25485 - DNA, 28 bp, synthetic construct
  source 1..28: mol_type = other DNA
gcgcgaggggaggagcgggaggaggcgg

SEQ ID NO: 25486 - DNA, 28 bp, synthetic construct
  source 1..28: mol_type = other DNA
cgaggggaggagcgggaggaggcggagg

SEQ ID NO: 25487 - DNA, 28 bp, synthetic construct
  source 1..28: mol_type = other DNA
agcgggaggaggcggaggatgttcccgg

SEQ ID NO: 25488 - DNA, 28 bp, synthetic construct
  source 1..28: mol_type = other DNA
gggaggaggcggaggatgttcccggcgg

SEQ ID NO: 25489 - DNA, 28 bp, synthetic construct
  source 1..28: mol_type = other DNA
aggcggaggatgttcccggcggctgcgg

SEQ ID NO: 25490 - DNA, 28 bp, synthetic construct
  source 1..28: mol_type = other DNA
ggaggatgttcccggcggctgcggccgg

SEQ ID NO: 25491 - DNA, 28 bp, synthetic construct
  source 1..28: mol_type = other DNA
gaggatgttcccggcggctgcggccggg

SEQ ID NO: 25492 - DNA, 28 bp, synthetic construct
  source 1..28: mol_type = other DNA
aggatgttcccggcggctgcggccgggg

SEQ ID NO: 25493 - DNA, 28 bp, synthetic construct
  source 1..28: mol_type = other DNA
ccgcgctgccccggccgcagccgccggg

SEQ ID NO: 25494 - DNA, 28 bp, synthetic construct
  source 1..28: mol_type = other DNA
ccggcggctgcggccggggcagcgcggg

SEQ ID NO: 25495 - DNA, 28 bp, synthetic construct
  source 1..28: mol_type = other DNA
ctgcggccggggcagcgcgggccagagg

SEQ ID NO: 25496 - DNA, 28 bp, synthetic construct
  source 1..28: mol_type = other DNA
gccggggcagcgcgggccagaggcgcgg

SEQ ID NO: 25497 - DNA, 28 bp, synthetic construct
  source 1..28: mol_type = other DNA
gccgcgcctctggcccgcgctgccccgg

SEQ ID NO: 25498 - DNA, 28 bp, synthetic construct
  source 1..28: mol_type = other DNA
cagcgcgggccagaggcgcggcgtgcgg

SEQ ID NO: 25499 - DNA, 28 bp, synthetic construct
  source 1..28: mol_type = other DNA
ccagaggcgcggcgtgcggagccctcgg

SEQ ID NO: 25500 - DNA, 28 bp, synthetic construct
  source 1..28: mol_type = other DNA
gcggcgtgcggagccctcggctgcccgg

SEQ ID NO: 25501 - DNA, 28 bp, synthetic construct
  source 1..28: mol_type = other DNA
gcgtgcggagccctcggctgcccggcgg

SEQ ID NO: 25502 - DNA, 28 bp, synthetic construct
  source 1..28: mol_type = other DNA
gagccctcggctgcccggcggagcgcgg

SEQ ID NO: 25503 - DNA, 28 bp, synthetic construct
  source 1..28: mol_type = other DNA
ccctcggctgcccggcggagcgcggcgg

SEQ ID NO: 25504 - DNA, 28 bp, synthetic construct
  source 1..28: mol_type = other DNA
gccgccgcgctccgccgggcagccgagg

SEQ ID NO: 25505 - DNA, 28 bp, synthetic construct
  source 1..28: mol_type = other DNA
tcggctgcccggcggagcgcggcggcgg

SEQ ID NO: 25506 - DNA, 28 bp, synthetic construct
  source 1..28: mol_type = other DNA
cggctgcccggcggagcgcggcggcggg

SEQ ID NO: 25507 - DNA, 28 bp, synthetic construct
  source 1..28: mol_type = other DNA
tgcccggcggagcgcggcggcgggctgg

SEQ ID NO: 25508 - DNA, 28 bp, synthetic construct
  source 1..28: mol_type = other DNA
cgccagcccgccgccgcgctccgccggg

SEQ ID NO: 25509 - DNA, 28 bp, synthetic construct
  source 1..28: mol_type = other DNA
ccgccagcccgccgccgcgctccgccgg

SEQ ID NO: 25510 - DNA, 28 bp, synthetic construct
  source 1..28: mol_type = other DNA
cggcggagcgcggcggcgggctggcggg

SEQ ID NO: 25511 - DNA, 28 bp, synthetic construct
  source 1..28: mol_type = other DNA
ggagcgcggcggcgggctggcgggaagg

SEQ ID NO: 25512 - DNA, 28 bp, synthetic construct
  source 1..28: mol_type = other DNA
gcggcggcgggctggcgggaaggcgcgg

SEQ ID NO: 25513 - DNA, 28 bp, synthetic construct
  source 1..28: mol_type = other DNA
cggcggcgggctggcgggaaggcgcggg

SEQ ID NO: 25514 - DNA, 28 bp, synthetic construct
  source 1..28: mol_type = other DNA
ggaaggcgcgggctttgcgctgcgccgg

SEQ ID NO: 25515 - DNA, 28 bp, synthetic construct
  source 1..28: mol_type = other DNA
gaaggcgcgggctttgcgctgcgccggg

SEQ ID NO: 25516 - DNA, 28 bp, synthetic construct
  source 1..28: mol_type = other DNA
aaggcgcgggctttgcgctgcgccgggg

SEQ ID NO: 25517 - DNA, 28 bp, synthetic construct
  source 1..28: mol_type = other DNA
cgccggggactctgaacccgagtcccgg

SEQ ID NO: 25518 - DNA, 28 bp, synthetic construct
  source 1..28: mol_type = other DNA
gccggggactctgaacccgagtcccggg

SEQ ID NO: 25519 - DNA, 28 bp, synthetic construct
  source 1..28: mol_type = other DNA
gcccgggactcgggttcagagtccccgg

SEQ ID NO: 25520 - DNA, 28 bp, synthetic construct
  source 1..28: mol_type = other DNA
gcgcaggagacaaagcccgggactcggg

SEQ ID NO: 25521 - DNA, 28 bp, synthetic construct
  source 1..28: mol_type = other DNA
agcgcaggagacaaagcccgggactcgg

SEQ ID NO: 25522 - DNA, 28 bp, synthetic construct
  source 1..28: mol_type = other DNA
gaaagcagcgcaggagacaaagcccggg

SEQ ID NO: 25523 - DNA, 28 bp, synthetic construct
  source 1..28: mol_type = other DNA
cgaaagcagcgcaggagacaaagcccgg

SEQ ID NO: 25524 - DNA, 28 bp, synthetic construct
  source 1..28: mol_type = other DNA
ggctttgtctcctgcgctgctttcgtgg

SEQ ID NO: 25525 - DNA, 28 bp, synthetic construct
  source 1..28: mol_type = other DNA
gtctcctgcgctgctttcgtggtgacgg

SEQ ID NO: 25526 - DNA, 28 bp, synthetic construct
  source 1..28: mol_type = other DNA
ctgaccgtcaccacgaaagcagcgcagg

SEQ ID NO: 25527 - DNA, 28 bp, synthetic construct
  source 1..28: mol_type = other DNA
ctgcgctgctttcgtggtgacggtcagg

SEQ ID NO: 25528 - DNA, 28 bp, synthetic construct
  source 1..28: mol_type = other DNA
tgcgctgctttcgtggtgacggtcaggg

SEQ ID NO: 25529 - DNA, 28 bp, synthetic construct
  source 1..28: mol_type = other DNA
gcgctgctttcgtggtgacggtcagggg

SEQ ID NO: 25530 - DNA, 28 bp, synthetic construct
  source 1..28: mol_type = other DNA
cgctgctttcgtggtgacggtcaggggg

SEQ ID NO: 25531 - DNA, 28 bp, synthetic construct
  source 1..28: mol_type = other DNA
ttcgtggtgacggtcagggggcgcccgg

SEQ ID NO: 25532 - DNA, 28 bp, synthetic construct
  source 1..28: mol_type = other DNA
tggtgacggtcagggggcgcccggtcgg

SEQ ID NO: 25533 - DNA, 28 bp, synthetic construct
  source 1..28: mol_type = other DNA
cggtcagggggcgcccggtcggcgaagg

SEQ ID NO: 25534 - DNA, 28 bp, synthetic construct
  source 1..28: mol_type = other DNA
ggtcagggggcgcccggtcggcgaaggg

SEQ ID NO: 25535 - DNA, 28 bp, synthetic construct
  source 1..28: mol_type = other DNA
gggggcgcccggtcggcgaagggcgcgg

SEQ ID NO: 25536 - DNA, 28 bp, synthetic construct
  source 1..28: mol_type = other DNA
ggggcgcccggtcggcgaagggcgcggg

SEQ ID NO: 25537 - DNA, 28 bp, synthetic construct
  source 1..28: mol_type = other DNA
cgcccggtcggcgaagggcgcgggccgg

SEQ ID NO: 25538 - DNA, 28 bp, synthetic construct
  source 1..28: mol_type = other DNA
gtccggcccgcgcccttcgccgaccggg

SEQ ID NO: 25539 - DNA, 28 bp, synthetic construct
  source 1..28: mol_type = other DNA
cgtccggcccgcgcccttcgccgaccgg

SEQ ID NO: 25540 - DNA, 28 bp, synthetic construct
  source 1..28: mol_type = other DNA
ggcgaagggcgcgggccggacgccgcgg

SEQ ID NO: 25541 - DNA, 28 bp, synthetic construct
  source 1..28: mol_type = other DNA
gcgaagggcgcgggccggacgccgcggg

SEQ ID NO: 25542 - DNA, 28 bp, synthetic construct
  source 1..28: mol_type = other DNA
cgaagggcgcgggccggacgccgcgggg

SEQ ID NO: 25543 - DNA, 28 bp, synthetic construct
  source 1..28: mol_type = other DNA
ggcgcgggccggacgccgcggggcttgg

SEQ ID NO: 25544 - DNA, 28 bp, synthetic construct
  source 1..28: mol_type = other DNA
gccggacgccgcggggcttggtccctgg

SEQ ID NO: 25545 - DNA, 28 bp, synthetic construct
  source 1..28: mol_type = other DNA
gccagggaccaagccccgcggcgtccgg

SEQ ID NO: 25546 - DNA, 28 bp, synthetic construct
  source 1..28: mol_type = other DNA
acgccgcggggcttggtccctggcccgg

SEQ ID NO: 25547 - DNA, 28 bp, synthetic construct
  source 1..28: mol_type = other DNA
cgtccgggccagggaccaagccccgcgg

SEQ ID NO: 25548 - DNA, 28 bp, synthetic construct
  source 1..28: mol_type = other DNA
ccttcagagcgcagcgtccgggccaggg

SEQ ID NO: 25549 - DNA, 28 bp, synthetic construct
  source 1..28: mol_type = other DNA
cctggcccggacgctgcgctctgaaggg

SEQ ID NO: 25550 - DNA, 28 bp, synthetic construct
  source 1..28: mol_type = other DNA
gcccggacgctgcgctctgaagggaagg

SEQ ID NO: 25551 - DNA, 28 bp, synthetic construct
  source 1..28: mol_type = other DNA
gccttcccttcagagcgcagcgtccggg

SEQ ID NO: 25552 - DNA, 28 bp, synthetic construct
  source 1..28: mol_type = other DNA
cgccttcccttcagagcgcagcgtccgg

SEQ ID NO: 25553 - DNA, 28 bp, synthetic construct
  source 1..28: mol_type = other DNA
gacgctgcgctctgaagggaaggcgcgg

SEQ ID NO: 25554 - DNA, 28 bp, synthetic construct
  source 1..28: mol_type = other DNA
gaagggaaggcgcggacgtgagtttcgg

SEQ ID NO: 25555 - DNA, 28 bp, synthetic construct
  source 1..28: mol_type = other DNA
tgagtttcggtgtgattgccttctgagg

SEQ ID NO: 25556 - DNA, 28 bp, synthetic construct
  source 1..28: mol_type = other DNA
gagtttcggtgtgattgccttctgaggg

SEQ ID NO: 25557 - DNA, 28 bp, synthetic construct
  source 1..28: mol_type = other DNA
agtttcggtgtgattgccttctgagggg

SEQ ID NO: 25558 - DNA, 28 bp, synthetic construct
  source 1..28: mol_type = other DNA
ttcggtgtgattgccttctgaggggagg

SEQ ID NO: 25559 - DNA, 28 bp, synthetic construct
  source 1..28: mol_type = other DNA
tcggtgtgattgccttctgaggggaggg

SEQ ID NO: 25560 - DNA, 28 bp, synthetic construct
  source 1..28: mol_type = other DNA
gattgccttctgaggggagggtctgtgg

SEQ ID NO: 25561 - DNA, 28 bp, synthetic construct
  source 1..28: mol_type = other DNA
attgccttctgaggggagggtctgtggg

SEQ ID NO: 25562 - DNA, 28 bp, synthetic construct
  source 1..28: mol_type = other DNA
tcatcccacagaccctcccctcagaagg

SEQ ID NO: 25563 - DNA, 28 bp, synthetic construct
  source 1..28: mol_type = other DNA
tctgaggggagggtctgtgggatgaagg

SEQ ID NO: 25564 - DNA, 28 bp, synthetic construct
  source 1..28: mol_type = other DNA
gaggggagggtctgtgggatgaaggcgg

SEQ ID NO: 25565 - DNA, 28 bp, synthetic construct
  source 1..28: mol_type = other DNA
gagggtctgtgggatgaaggcggcgcgg

SEQ ID NO: 25566 - DNA, 28 bp, synthetic construct
  source 1..28: mol_type = other DNA
gggatgaaggcggcgcggcgcgcaccgg

SEQ ID NO: 25567 - DNA, 28 bp, synthetic construct
  source 1..28: mol_type = other DNA
gcgcgcaccggtgtcgcctagcctgcgg

SEQ ID NO: 25568 - DNA, 28 bp, synthetic construct
  source 1..28: mol_type = other DNA
actaggtccgcaggctaggcgacaccgg

SEQ ID NO: 25569 - DNA, 28 bp, synthetic construct
  source 1..28: mol_type = other DNA
aggtctacaactaggtccgcaggctagg

SEQ ID NO: 25570 - DNA, 28 bp, synthetic construct
  source 1..28: mol_type = other DNA
ctgcaaggtctacaactaggtccgcagg

SEQ ID NO: 25571 - DNA, 28 bp, synthetic construct
  source 1..28: mol_type = other DNA
ctgcggacctagttgtagaccttgcagg

SEQ ID NO: 25572 - DNA, 28 bp, synthetic construct
  source 1..28: mol_type = other DNA
gcgaacgcctgcaaggtctacaactagg

SEQ ID NO: 25573 - DNA, 28 bp, synthetic construct
  source 1..28: mol_type = other DNA
gagggcgacgaagcgaacgcctgcaagg

SEQ ID NO: 25574 - DNA, 28 bp, synthetic construct
  source 1..28: mol_type = other DNA
ctctaaatggggagggggcggcggaggg

SEQ ID NO: 25575 - DNA, 28 bp, synthetic construct
  source 1..28: mol_type = other DNA
tctctaaatggggagggggcggcggagg

SEQ ID NO: 25576 - DNA, 28 bp, synthetic construct
  source 1..28: mol_type = other DNA
acatctctaaatggggagggggcggcgg

SEQ ID NO: 25577 - DNA, 28 bp, synthetic construct
  source 1..28: mol_type = other DNA
tgcacatctctaaatggggagggggcgg

SEQ ID NO: 25578 - DNA, 28 bp, synthetic construct
  source 1..28: mol_type = other DNA
aggtgcacatctctaaatggggaggggg

SEQ ID NO: 25579 - DNA, 28 bp, synthetic construct
  source 1..28: mol_type = other DNA
gaggtgcacatctctaaatggggagggg

SEQ ID NO: 25580 - DNA, 28 bp, synthetic construct
  source 1..28: mol_type = other DNA
tgaggtgcacatctctaaatggggaggg

SEQ ID NO: 25581 - DNA, 28 bp, synthetic construct
  source 1..28: mol_type = other DNA
gtgaggtgcacatctctaaatggggagg

SEQ ID NO: 25582 - DNA, 28 bp, synthetic construct
  source 1..28: mol_type = other DNA
tccccatttagagatgtgcacctcacgg

SEQ ID NO: 25583 - DNA, 28 bp, synthetic construct
  source 1..28: mol_type = other DNA
accgtgaggtgcacatctctaaatgggg

SEQ ID NO: 25584 - DNA, 28 bp, synthetic construct
  source 1..28: mol_type = other DNA
caccgtgaggtgcacatctctaaatggg

SEQ ID NO: 25585 - DNA, 28 bp, synthetic construct
  source 1..28: mol_type = other DNA
acaccgtgaggtgcacatctctaaatgg

SEQ ID NO: 25586 - DNA, 28 bp, synthetic construct
  source 1..28: mol_type = other DNA
gaacttctctgaggtgcacaccgtgagg

SEQ ID NO: 25587 - DNA, 28 bp, synthetic construct
  source 1..28: mol_type = other DNA
cacctcagagaagttctgtctgattcgg

SEQ ID NO: 25588 - DNA, 28 bp, synthetic construct
  source 1..28: mol_type = other DNA
caccgaatcagacagaacttctctgagg

SEQ ID NO: 25589 - DNA, 28 bp, synthetic construct
  source 1..28: mol_type = other DNA
cagagaagttctgtctgattcggtgcgg

SEQ ID NO: 25590 - DNA, 28 bp, synthetic construct
  source 1..28: mol_type = other DNA
gttctgtctgattcggtgcggcgtgcgg

SEQ ID NO: 25591 - DNA, 28 bp, synthetic construct
  source 1..28: mol_type = other DNA
gtctgattcggtgcggcgtgcggtacgg

SEQ ID NO: 25592 - DNA, 28 bp, synthetic construct
  source 1..28: mol_type = other DNA
tctgattcggtgcggcgtgcggtacggg

SEQ ID NO: 25593 - DNA, 28 bp, synthetic construct
  source 1..28: mol_type = other DNA
ttcggtgcggcgtgcggtacgggagcgg

SEQ ID NO: 25594 - DNA, 28 bp, synthetic construct
  source 1..28: mol_type = other DNA
tcggtgcggcgtgcggtacgggagcggg

SEQ ID NO: 25595 - DNA, 28 bp, synthetic construct
  source 1..28: mol_type = other DNA
gtgcggcgtgcggtacgggagcgggagg

SEQ ID NO: 25596 - DNA, 28 bp, synthetic construct
  source 1..28: mol_type = other DNA
tgcggcgtgcggtacgggagcgggaggg

SEQ ID NO: 25597 - DNA, 28 bp, synthetic construct
  source 1..28: mol_type = other DNA
ggcgtgcggtacgggagcgggagggagg

SEQ ID NO: 25598 - DNA, 28 bp, synthetic construct
  source 1..28: mol_type = other DNA
gcgtgcggtacgggagcgggagggaggg

SEQ ID NO: 25599 - DNA, 28 bp, synthetic construct
  source 1..28: mol_type = other DNA
gtacgggagcgggagggagggagcacgg

SEQ ID NO: 25600 - DNA, 28 bp, synthetic construct
  source 1..28: mol_type = other DNA
tacgggagcgggagggagggagcacggg

SEQ ID NO: 25601 - DNA, 28 bp, synthetic construct
  source 1..28: mol_type = other DNA
gggagcgggagggagggagcacgggcgg

SEQ ID NO: 25602 - DNA, 28 bp, synthetic construct
  source 1..28: mol_type = other DNA
gcacgggcggagagagcgccagagccgg

SEQ ID NO: 25603 - DNA, 28 bp, synthetic construct
  source 1..28: mol_type = other DNA
cacgggcggagagagcgccagagccggg

SEQ ID NO: 25604 - DNA, 28 bp, synthetic construct
  source 1..28: mol_type = other DNA
gcgccagagccgggccgagccgcgctgg

SEQ ID NO: 25605 - DNA, 28 bp, synthetic construct
  source 1..28: mol_type = other DNA
actccagcgcggctcggcccggctctgg

SEQ ID NO: 25606 - DNA, 28 bp, synthetic construct
  source 1..28: mol_type = other DNA
tttgtaactccagcgcggctcggcccgg

SEQ ID NO: 25607 - DNA, 28 bp, synthetic construct
  source 1..28: mol_type = other DNA
tagagtttgtaactccagcgcggctcgg

SEQ ID NO: 25608 - DNA, 28 bp, synthetic construct
  source 1..28: mol_type = other DNA
cacaatagagtttgtaactccagcgcgg

SEQ ID NO: 25609 - DNA, 28 bp, synthetic construct
  source 1..28: mol_type = other DNA
attgtgacgcacttactacgactgacgg

SEQ ID NO: 25610 - DNA, 28 bp, synthetic construct
  source 1..28: mol_type = other DNA
agcaagtctggggaaggtctggcagcgg

SEQ ID NO: 25611 - DNA, 28 bp, synthetic construct
  source 1..28: mol_type = other DNA
gagggcagcaagtctggggaaggtctgg

SEQ ID NO: 25612 - DNA, 28 bp, synthetic construct
  source 1..28: mol_type = other DNA
atgctgagggcagcaagtctggggaagg

SEQ ID NO: 25613 - DNA, 28 bp, synthetic construct
  source 1..28: mol_type = other DNA
gaaaatgctgagggcagcaagtctgggg

SEQ ID NO: 25614 - DNA, 28 bp, synthetic construct
  source 1..28: mol_type = other DNA
cgaaaatgctgagggcagcaagtctggg

SEQ ID NO: 25615 - DNA, 28 bp, synthetic construct
  source 1..28: mol_type = other DNA
ccagacttgctgccctcagcattttcgg

SEQ ID NO: 25616 - DNA, 28 bp, synthetic construct
  source 1..28: mol_type = other DNA
tgccctcagcattttcggcaaacaatgg

SEQ ID NO: 25617 - DNA, 28 bp, synthetic construct
  source 1..28: mol_type = other DNA
gccctcagcattttcggcaaacaatggg

SEQ ID NO: 25618 - DNA, 28 bp, synthetic construct
  source 1..28: mol_type = other DNA
ccctcagcattttcggcaaacaatgggg

SEQ ID NO: 25619 - DNA, 28 bp, synthetic construct
  source 1..28: mol_type = other DNA
gccccattgtttgccgaaaatgctgagg

SEQ ID NO: 25620 - DNA, 28 bp, synthetic construct
  source 1..28: mol_type = other DNA
cagcattttcggcaaacaatggggccgg

SEQ ID NO: 25621 - DNA, 28 bp, synthetic construct
  source 1..28: mol_type = other DNA
tttcggcaaacaatggggccggagcagg

SEQ ID NO: 25622 - DNA, 28 bp, synthetic construct
  source 1..28: mol_type = other DNA
ttcggcaaacaatggggccggagcaggg

SEQ ID NO: 25623 - DNA, 28 bp, synthetic construct
  source 1..28: mol_type = other DNA
aacaatggggccggagcagggaacgcgg

SEQ ID NO: 25624 - DNA, 28 bp, synthetic construct
  source 1..28: mol_type = other DNA
aggcggctggccgcgttccctgctccgg

SEQ ID NO: 25625 - DNA, 28 bp, synthetic construct
  source 1..28: mol_type = other DNA
cgcagatgcagcgattgcaggcggctgg

SEQ ID NO: 25626 - DNA, 28 bp, synthetic construct
  source 1..28: mol_type = other DNA
cgggcgcagatgcagcgattgcaggcgg

SEQ ID NO: 25627 - DNA, 28 bp, synthetic construct
  source 1..28: mol_type = other DNA
gagcgggcgcagatgcagcgattgcagg

SEQ ID NO: 25628 - DNA, 28 bp, synthetic construct
  source 1..28: mol_type = other DNA
tgcatctgcgcccgctcctgtgctccgg

SEQ ID NO: 25629 - DNA, 28 bp, synthetic construct
  source 1..28: mol_type = other DNA
aggtaggacgccggagcacaggagcggg

SEQ ID NO: 25630 - DNA, 28 bp, synthetic construct
  source 1..28: mol_type = other DNA
taggtaggacgccggagcacaggagcgg

SEQ ID NO: 25631 - DNA, 28 bp, synthetic construct
  source 1..28: mol_type = other DNA
ggggttaggtaggacgccggagcacagg

SEQ ID NO: 25632 - DNA, 28 bp, synthetic construct
  source 1..28: mol_type = other DNA
tgtgctccggcgtcctacctaaccccgg

SEQ ID NO: 25633 - DNA, 28 bp, synthetic construct
  source 1..28: mol_type = other DNA
gtgctccggcgtcctacctaaccccggg

SEQ ID NO: 25634 - DNA, 28 bp, synthetic construct
  source 1..28: mol_type = other DNA
gacttcccggggttaggtaggacgccgg

SEQ ID NO: 25635 - DNA, 28 bp, synthetic construct
  source 1..28: mol_type = other DNA
cggctctgacttcccggggttaggtagg

SEQ ID NO: 25636 - DNA, 28 bp, synthetic construct
  source 1..28: mol_type = other DNA
ccagcggctctgacttcccggggttagg

SEQ ID NO: 25637 - DNA, 28 bp, synthetic construct
  source 1..28: mol_type = other DNA
ctaaccccgggaagtcagagccgctggg

SEQ ID NO: 25638 - DNA, 28 bp, synthetic construct
  source 1..28: mol_type = other DNA
aactcccagcggctctgacttcccgggg

SEQ ID NO: 25639 - DNA, 28 bp, synthetic construct
  source 1..28: mol_type = other DNA
aaactcccagcggctctgacttcccggg

SEQ ID NO: 25640 - DNA, 28 bp, synthetic construct
  source 1..28: mol_type = other DNA
gaaactcccagcggctctgacttcccgg

SEQ ID NO: 25641 - DNA, 28 bp, synthetic construct
  source 1..28: mol_type = other DNA
cttcgagtaagtcagaaactcccagcgg

SEQ ID NO: 25642 - DNA, 28 bp, synthetic construct
  source 1..28: mol_type = other DNA
ctgacttactcgaagaagtctgtcctgg

SEQ ID NO: 25643 - DNA, 28 bp, synthetic construct
  source 1..28: mol_type = other DNA
tgacttactcgaagaagtctgtcctggg

SEQ ID NO: 25644 - DNA, 28 bp, synthetic construct
  source 1..28: mol_type = other DNA
gtctattcgtgtgtgctctttgcccagg

SEQ ID NO: 25645 - DNA, 28 bp, synthetic construct
  source 1..28: mol_type = other DNA
atagacttcagattagctgcttctctgg

SEQ ID NO: 25646 - DNA, 28 bp, synthetic construct
  source 1..28: mol_type = other DNA
taacaatgtcaacagcttgcggaactgg

SEQ ID NO: 25647 - DNA, 28 bp, synthetic construct
  source 1..28: mol_type = other DNA
atacagtaacaatgtcaacagcttgcgg

SEQ ID NO: 25648 - DNA, 28 bp, synthetic construct
  source 1..28: mol_type = other DNA
gttgacattgttactgtattttgtttgg

SEQ ID NO: 25649 - DNA, 28 bp, synthetic construct
  source 1..28: mol_type = other DNA
ttgacattgttactgtattttgtttggg

SEQ ID NO: 25650 - DNA, 28 bp, synthetic construct
  source 1..28: mol_type = other DNA
tgacattgttactgtattttgtttgggg

SEQ ID NO: 25651 - DNA, 28 bp, synthetic construct
  source 1..28: mol_type = other DNA
gacattgttactgtattttgtttggggg

SEQ ID NO: 25652 - DNA, 28 bp, synthetic construct
  source 1..28: mol_type = other DNA
aaaggtgtaatttttttttggtagaggg

SEQ ID NO: 25653 - DNA, 28 bp, synthetic construct
  source 1..28: mol_type = other DNA
taaaggtgtaatttttttttggtagagg

SEQ ID NO: 25654 - DNA, 28 bp, synthetic construct
  source 1..28: mol_type = other DNA
aaataataaaggtgtaatttttttttgg

SEQ ID NO: 25655 - DNA, 28 bp, synthetic construct
  source 1..28: mol_type = other DNA
aaaaaaattacacctttattattttagg

SEQ ID NO: 25656 - DNA, 28 bp, synthetic construct
  source 1..28: mol_type = other DNA
aaaaaaattgcacctaaaataataaagg

SEQ ID NO: 25657 - DNA, 28 bp, synthetic construct
  source 1..28: mol_type = other DNA
ttattttaggtgcaatttttttatttgg

SEQ ID NO: 25658 - DNA, 28 bp, synthetic construct
  source 1..28: mol_type = other DNA
tattttaggtgcaatttttttatttggg

SEQ ID NO: 25659 - DNA, 28 bp, synthetic construct
  source 1..28: mol_type = other DNA
ttaaccctaagaatttttaatcgctagg

SEQ ID NO: 25660 - DNA, 28 bp, synthetic construct
  source 1..28: mol_type = other DNA
ctcacctagcgattaaaaattcttaggg

SEQ ID NO: 25661 - DNA, 28 bp, synthetic construct
  source 1..28: mol_type = other DNA
tctcacctagcgattaaaaattcttagg

SEQ ID NO: 25662 - DNA, 28 bp, synthetic construct
  source 1..28: mol_type = other DNA
tttacttgcagaaaaaaagaccaaatgg

SEQ ID NO: 25663 - DNA, 28 bp, synthetic construct
  source 1..28: mol_type = other DNA
gacagctgcccccacggcagccctcagg

SEQ ID NO: 25664 - DNA, 28 bp, synthetic construct
  source 1..28: mol_type = other DNA
acagctgcccccacggcagccctcaggg

SEQ ID NO: 25665 - DNA, 28 bp, synthetic construct
  source 1..28: mol_type = other DNA
cagcgggccctgagggctgccgtggggg

SEQ ID NO: 25666 - DNA, 28 bp, synthetic construct
  source 1..28: mol_type = other DNA
ccagcgggccctgagggctgccgtgggg

SEQ ID NO: 25667 - DNA, 28 bp, synthetic construct
  source 1..28: mol_type = other DNA
gccagcgggccctgagggctgccgtggg

SEQ ID NO: 25668 - DNA, 28 bp, synthetic construct
  source 1..28: mol_type = other DNA
ggccagcgggccctgagggctgccgtgg

SEQ ID NO: 25669 - DNA, 28 bp, synthetic construct
  source 1..28: mol_type = other DNA
ggcaggtggggccagcgggccctgaggg

SEQ ID NO: 25670 - DNA, 28 bp, synthetic construct
  source 1..28: mol_type = other DNA
tggcaggtggggccagcgggccctgagg

SEQ ID NO: 25671 - DNA, 28 bp, synthetic construct
  source 1..28: mol_type = other DNA
gcccgctggccccacctgccagccctgg

SEQ ID NO: 25672 - DNA, 28 bp, synthetic construct
  source 1..28: mol_type = other DNA
gccagggctggcaggtggggccagcggg

SEQ ID NO: 25673 - DNA, 28 bp, synthetic construct
  source 1..28: mol_type = other DNA
ggccagggctggcaggtggggccagcgg

SEQ ID NO: 25674 - DNA, 28 bp, synthetic construct
  source 1..28: mol_type = other DNA
gcaaaagggccagggctggcaggtgggg

SEQ ID NO: 25675 - DNA, 28 bp, synthetic construct
  source 1..28: mol_type = other DNA
agcaaaagggccagggctggcaggtggg

SEQ ID NO: 25676 - DNA, 28 bp, synthetic construct
  source 1..28: mol_type = other DNA
tagcaaaagggccagggctggcaggtgg

SEQ ID NO: 25677 - DNA, 28 bp, synthetic construct
  source 1..28: mol_type = other DNA
tggtagcaaaagggccagggctggcagg

SEQ ID NO: 25678 - DNA, 28 bp, synthetic construct
  source 1..28: mol_type = other DNA
gatctggtagcaaaagggccagggctgg

SEQ ID NO: 25679 - DNA, 28 bp, synthetic construct
  source 1..28: mol_type = other DNA
cggggatctggtagcaaaagggccaggg

SEQ ID NO: 25680 - DNA, 28 bp, synthetic construct
  source 1..28: mol_type = other DNA
gcggggatctggtagcaaaagggccagg

SEQ ID NO: 25681 - DNA, 28 bp, synthetic construct
  source 1..28: mol_type = other DNA
gaaaagcggggatctggtagcaaaaggg

SEQ ID NO: 25682 - DNA, 28 bp, synthetic construct
  source 1..28: mol_type = other DNA
tgaaaagcggggatctggtagcaaaagg

SEQ ID NO: 25683 - DNA, 28 bp, synthetic construct
  source 1..28: mol_type = other DNA
ctcataaagatgaaaagcggggatctgg

SEQ ID NO: 25684 - DNA, 28 bp, synthetic construct
  source 1..28: mol_type = other DNA
gatcttctcataaagatgaaaagcgggg

SEQ ID NO: 25685 - DNA, 28 bp, synthetic construct
  source 1..28: mol_type = other DNA
ggatcttctcataaagatgaaaagcggg

SEQ ID NO: 25686 - DNA, 28 bp, synthetic construct
  source 1..28: mol_type = other DNA
aggatcttctcataaagatgaaaagcgg

SEQ ID NO: 25687 - DNA, 28 bp, synthetic construct
  source 1..28: mol_type = other DNA
ctcagtgcaatgggtaagcaatgcctgg

SEQ ID NO: 25688 - DNA, 28 bp, synthetic construct
  source 1..28: mol_type = other DNA
tcagtgcaatgggtaagcaatgcctggg

SEQ ID NO: 25689 - DNA, 28 bp, synthetic construct
  source 1..28: mol_type = other DNA
aatgggtaagcaatgcctgggtaagagg

SEQ ID NO: 25690 - DNA, 28 bp, synthetic construct
  source 1..28: mol_type = other DNA
gcctgggtaagaggcagttgacgtgtgg

SEQ ID NO: 25691 - DNA, 28 bp, synthetic construct
  source 1..28: mol_type = other DNA
tccacacgtcaactgcctcttacccagg

SEQ ID NO: 25692 - DNA, 28 bp, synthetic construct
  source 1..28: mol_type = other DNA
gggtaagaggcagttgacgtgtggatgg

SEQ ID NO: 25693 - DNA, 28 bp, synthetic construct
  source 1..28: mol_type = other DNA
cgtgtggatggttgaatctgcttgaagg

SEQ ID NO: 25694 - DNA, 28 bp, synthetic construct
  source 1..28: mol_type = other DNA
gttgaatctgcttgaaggctgtgtgtgg

SEQ ID NO: 25695 - DNA, 28 bp, synthetic construct
  source 1..28: mol_type = other DNA
taaatcagttacggggttttaaaagggg

SEQ ID NO: 25696 - DNA, 28 bp, synthetic construct
  source 1..28: mol_type = other DNA
ataaatcagttacggggttttaaaaggg

SEQ ID NO: 25697 - DNA, 28 bp, synthetic construct
  source 1..28: mol_type = other DNA
aataaatcagttacggggttttaaaagg

SEQ ID NO: 25698 - DNA, 28 bp, synthetic construct
  source 1..28: mol_type = other DNA
ctaaagatggaataaatcagttacgggg

SEQ ID NO: 25699 - DNA, 28 bp, synthetic construct
  source 1..28: mol_type = other DNA
tctaaagatggaataaatcagttacggg

SEQ ID NO: 25700 - DNA, 28 bp, synthetic construct
  source 1..28: mol_type = other DNA
atctaaagatggaataaatcagttacgg

SEQ ID NO: 25701 - DNA, 28 bp, synthetic construct
  source 1..28: mol_type = other DNA
gtaactgatttattccatctttagatgg

SEQ ID NO: 25702 - DNA, 28 bp, synthetic construct
  source 1..28: mol_type = other DNA
taactgatttattccatctttagatggg

SEQ ID NO: 25703 - DNA, 28 bp, synthetic construct
  source 1..28: mol_type = other DNA
ggaaccatcatgctgttctccatagagg

SEQ ID NO: 25704 - DNA, 28 bp, synthetic construct
  source 1..28: mol_type = other DNA
acagcctctatggagaacagcatgatgg

SEQ ID NO: 25705 - DNA, 28 bp, synthetic construct
  source 1..28: mol_type = other DNA
ggaatgtaaaatggcacagcctctatgg

SEQ ID NO: 25706 - DNA, 28 bp, synthetic construct
  source 1..28: mol_type = other DNA
tgtgccattttacattcccaccaacagg

SEQ ID NO: 25707 - DNA, 28 bp, synthetic construct
  source 1..28: mol_type = other DNA
gtgccattttacattcccaccaacaggg

SEQ ID NO: 25708 - DNA, 28 bp, synthetic construct
  source 1..28: mol_type = other DNA
gtgccctgttggtgggaatgtaaaatgg

SEQ ID NO: 25709 - DNA, 28 bp, synthetic construct
  source 1..28: mol_type = other DNA
tttacattcccaccaacagggcacaagg

SEQ ID NO: 25710 - DNA, 28 bp, synthetic construct
  source 1..28: mol_type = other DNA
ttacattcccaccaacagggcacaaggg

SEQ ID NO: 25711 - DNA, 28 bp, synthetic construct
  source 1..28: mol_type = other DNA
actggaacccttgtgccctgttggtggg

SEQ ID NO: 25712 - DNA, 28 bp, synthetic construct
  source 1..28: mol_type = other DNA
aactggaacccttgtgccctgttggtgg

SEQ ID NO: 25713 - DNA, 28 bp, synthetic construct
  source 1..28: mol_type = other DNA
agaaactggaacccttgtgccctgttgg

SEQ ID NO: 25714 - DNA, 28 bp, synthetic construct
  source 1..28: mol_type = other DNA
agtgttggtaagtatgtggagaaactgg

SEQ ID NO: 25715 - DNA, 28 bp, synthetic construct
  source 1..28: mol_type = other DNA
aaaaaaaaaagtgttggtaagtatgtgg

SEQ ID NO: 25716 - DNA, 28 bp, synthetic construct
  source 1..28: mol_type = other DNA
gttaaaaaaaaaaaaaaaaaagtgttgg

SEQ ID NO: 25717 - DNA, 28 bp, synthetic construct
  source 1..28: mol_type = other DNA
cactgtgctttggatttatatttactgg

SEQ ID NO: 25718 - DNA, 28 bp, synthetic construct
  source 1..28: mol_type = other DNA
ttatatttactggcttagatttgtatgg

SEQ ID NO: 25719 - DNA, 28 bp, synthetic construct
  source 1..28: mol_type = other DNA
ttgttctgtatcttgactatggtggtgg

SEQ ID NO: 25720 - DNA, 28 bp, synthetic construct
  source 1..28: mol_type = other DNA
gagttgttctgtatcttgactatggtgg

SEQ ID NO: 25721 - DNA, 28 bp, synthetic construct
  source 1..28: mol_type = other DNA
gttgagttgttctgtatcttgactatgg

SEQ ID NO: 25722 - DNA, 28 bp, synthetic construct
  source 1..28: mol_type = other DNA
caagatacagaacaactcaaccacaagg

SEQ ID NO: 25723 - DNA, 28 bp, synthetic construct
  source 1..28: mol_type = other DNA
aaaaaggtatcatgagaaatccttgtgg

SEQ ID NO: 25724 - DNA, 28 bp, synthetic construct
  source 1..28: mol_type = other DNA
gagagaggtggctgtggctataaaaagg

SEQ ID NO: 25725 - DNA, 28 bp, synthetic construct
  source 1..28: mol_type = other DNA
caaggaagagggagagaggtggctgtgg

SEQ ID NO: 25726 - DNA, 28 bp, synthetic construct
  source 1..28: mol_type = other DNA
aatgctcaaggaagagggagagaggtgg

SEQ ID NO: 25727 - DNA, 28 bp, synthetic construct
  source 1..28: mol_type = other DNA
caaaatgctcaaggaagagggagagagg

SEQ ID NO: 25728 - DNA, 28 bp, synthetic construct
  source 1..28: mol_type = other DNA
catatgacaaaatgctcaaggaagaggg

SEQ ID NO: 25729 - DNA, 28 bp, synthetic construct
  source 1..28: mol_type = other DNA
cctcttccttgagcattttgtcatatgg

SEQ ID NO: 25730 - DNA, 28 bp, synthetic construct
  source 1..28: mol_type = other DNA
caatgaccatatgacaaaatgctcaagg

SEQ ID NO: 25731 - DNA, 28 bp, synthetic construct
  source 1..28: mol_type = other DNA
cttgagcattttgtcatatggtcattgg

SEQ ID NO: 25732 - DNA, 28 bp, synthetic construct
  source 1..28: mol_type = other DNA
acatgcaaacacagtgtccttcaacagg

SEQ ID NO: 25733 - DNA, 28 bp, synthetic construct
  source 1..28: mol_type = other DNA
tgaaggacactgtgtttgcatgttctgg

SEQ ID NO: 25734 - DNA, 28 bp, synthetic construct
  source 1..28: mol_type = other DNA
gacactgtgtttgcatgttctggcaagg

SEQ ID NO: 25735 - DNA, 28 bp, synthetic construct
  source 1..28: mol_type = other DNA
gtgtttgcatgttctggcaaggccctgg

SEQ ID NO: 25736 - DNA, 28 bp, synthetic construct
  source 1..28: mol_type = other DNA
tgttctggcaaggccctggcacagctgg

SEQ ID NO: 25737 - DNA, 28 bp, synthetic construct
  source 1..28: mol_type = other DNA
caaggccctggcacagctggaactcagg

SEQ ID NO: 25738 - DNA, 28 bp, synthetic construct
  source 1..28: mol_type = other DNA
aaggccctggcacagctggaactcaggg

SEQ ID NO: 25739 - DNA, 28 bp, synthetic construct
  source 1..28: mol_type = other DNA
gccctggcacagctggaactcagggagg

SEQ ID NO: 25740 - DNA, 28 bp, synthetic construct
  source 1..28: mol_type = other DNA
tcctccctgagttccagctgtgccaggg

SEQ ID NO: 25741 - DNA, 28 bp, synthetic construct
  source 1..28: mol_type = other DNA
atcctccctgagttccagctgtgccagg

SEQ ID NO: 25742 - DNA, 28 bp, synthetic construct
  source 1..28: mol_type = other DNA
aggctggagtgcactggtgcgatcttgg

SEQ ID NO: 25743 - DNA, 28 bp, synthetic construct
  source 1..28: mol_type = other DNA
gcaacctccaactcccaagttcaagcgg

SEQ ID NO: 25744 - DNA, 28 bp, synthetic construct
  source 1..28: mol_type = other DNA
agaaccgcttgaacttgggagttggagg

SEQ ID NO: 25745 - DNA, 28 bp, synthetic construct
  source 1..28: mol_type = other DNA
aggagaaccgcttgaacttgggagttgg

SEQ ID NO: 25746 - DNA, 28 bp, synthetic construct
  source 1..28: mol_type = other DNA
tgaggcaggagaaccgcttgaacttggg

SEQ ID NO: 25747 - DNA, 28 bp, synthetic construct
  source 1..28: mol_type = other DNA
ctgaggcaggagaaccgcttgaacttgg

SEQ ID NO: 25748 - DNA, 28 bp, synthetic construct
  source 1..28: mol_type = other DNA
ctcctgcctcagcctcccaagtagctgg

SEQ ID NO: 25749 - DNA, 28 bp, synthetic construct
  source 1..28: mol_type = other DNA
tcctgcctcagcctcccaagtagctggg

SEQ ID NO: 25750 - DNA, 28 bp, synthetic construct
  source 1..28: mol_type = other DNA
tcccagctacttgggaggctgaggcagg

SEQ ID NO: 25751 - DNA, 28 bp, synthetic construct
  source 1..28: mol_type = other DNA
gtaatcccagctacttgggaggctgagg

SEQ ID NO: 25752 - DNA, 28 bp, synthetic construct
  source 1..28: mol_type = other DNA
cagcctcccaagtagctgggattacagg

SEQ ID NO: 25753 - DNA, 28 bp, synthetic construct
  source 1..28: mol_type = other DNA
gtgcctgtaatcccagctacttgggagg

SEQ ID NO: 25754 - DNA, 28 bp, synthetic construct
  source 1..28: mol_type = other DNA
tacgtgcctgtaatcccagctacttggg

SEQ ID NO: 25755 - DNA, 28 bp, synthetic construct
  source 1..28: mol_type = other DNA
gtacgtgcctgtaatcccagctacttgg

SEQ ID NO: 25756 - DNA, 28 bp, synthetic construct
  source 1..28: mol_type = other DNA
aaatacaaaaattagctgggtgtggtgg

SEQ ID NO: 25757 - DNA, 28 bp, synthetic construct
  source 1..28: mol_type = other DNA
taaaaatacaaaaattagctgggtgtgg

SEQ ID NO: 25758 - DNA, 28 bp, synthetic construct
  source 1..28: mol_type = other DNA
tctaataaaaatacaaaaattagctggg

SEQ ID NO: 25759 - DNA, 28 bp, synthetic construct
  source 1..28: mol_type = other DNA
ctctaataaaaatacaaaaattagctgg

SEQ ID NO: 25760 - DNA, 28 bp, synthetic construct
  source 1..28: mol_type = other DNA
ctaatttttgtatttttattagagatgg

SEQ ID NO: 25761 - DNA, 28 bp, synthetic construct
  source 1..28: mol_type = other DNA
taatttttgtatttttattagagatggg

SEQ ID NO: 25762 - DNA, 28 bp, synthetic construct
  source 1..28: mol_type = other DNA
ttattagagatgggtttcaccatgttgg

SEQ ID NO: 25763 - DNA, 28 bp, synthetic construct
  source 1..28: mol_type = other DNA
agagatgggtttcaccatgttggccagg

SEQ ID NO: 25764 - DNA, 28 bp, synthetic construct
  source 1..28: mol_type = other DNA
atgggtttcaccatgttggccaggctgg

SEQ ID NO: 25765 - DNA, 28 bp, synthetic construct
  source 1..28: mol_type = other DNA
gagttcgagaccagcctggccaacatgg

SEQ ID NO: 25766 - DNA, 28 bp, synthetic construct
  source 1..28: mol_type = other DNA
tgaggtcaggagttcgagaccagcctgg

SEQ ID NO: 25767 - DNA, 28 bp, synthetic construct
  source 1..28: mol_type = other DNA
aggctggtctcgaactcctgacctcagg

SEQ ID NO: 25768 - DNA, 28 bp, synthetic construct
  source 1..28: mol_type = other DNA
caaggcgggcagatcacctgaggtcagg

SEQ ID NO: 25769 - DNA, 28 bp, synthetic construct
  source 1..28: mol_type = other DNA
ctgacctcaggtgatctgcccgccttgg

SEQ ID NO: 25770 - DNA, 28 bp, synthetic construct
  source 1..28: mol_type = other DNA
gaggccaaggcgggcagatcacctgagg

SEQ ID NO: 25771 - DNA, 28 bp, synthetic construct
  source 1..28: mol_type = other DNA
tgcccgccttggcctcccaaagtgttgg

SEQ ID NO: 25772 - DNA, 28 bp, synthetic construct
  source 1..28: mol_type = other DNA
gcccgccttggcctcccaaagtgttggg

SEQ ID NO: 25773 - DNA, 28 bp, synthetic construct
  source 1..28: mol_type = other DNA
tcttcattagcacaagtgcaagttaagg

SEQ ID NO: 25774 - DNA, 28 bp, synthetic construct
  source 1..28: mol_type = other DNA
tttgtcacagaaggaaaagaacaggagg

SEQ ID NO: 25775 - DNA, 28 bp, synthetic construct
  source 1..28: mol_type = other DNA
tgttttgtcacagaaggaaaagaacagg

SEQ ID NO: 25776 - DNA, 28 bp, synthetic construct
  source 1..28: mol_type = other DNA
gacagataacttgttttgtcacagaagg

SEQ ID NO: 25777 - DNA, 28 bp, synthetic construct
  source 1..28: mol_type = other DNA
tctgtgacaaaacaagttatctgtctgg

SEQ ID NO: 25778 - DNA, 28 bp, synthetic construct
  source 1..28: mol_type = other DNA
ctgtgacaaaacaagttatctgtctggg

SEQ ID NO: 25779 - DNA, 28 bp, synthetic construct
  source 1..28: mol_type = other DNA
aacaagttatctgtctgggaagacatgg

SEQ ID NO: 25780 - DNA, 28 bp, synthetic construct
  source 1..28: mol_type = other DNA
accttgattttgctaaccacttgagtgg

SEQ ID NO: 25781 - DNA, 28 bp, synthetic construct
  source 1..28: mol_type = other DNA
gaaaagtttttctttttattcaaaatgg

SEQ ID NO: 25782 - DNA, 28 bp, synthetic construct
  source 1..28: mol_type = other DNA
aaaagtttttctttttattcaaaatggg

SEQ ID NO: 25783 - DNA, 28 bp, synthetic construct
  source 1..28: mol_type = other DNA
aagcttctcacttaaaagtcacaaaagg

SEQ ID NO: 25784 - DNA, 28 bp, synthetic construct
  source 1..28: mol_type = other DNA
atatgattattgataacacactgtaggg

SEQ ID NO: 25785 - DNA, 28 bp, synthetic construct
  source 1..28: mol_type = other DNA
gatatgattattgataacacactgtagg

SEQ ID NO: 25786 - DNA, 28 bp, synthetic construct
  source 1..28: mol_type = other DNA
ttatttctgagaaccgtcagagttgagg

SEQ ID NO: 25787 - DNA, 28 bp, synthetic construct
  source 1..28: mol_type = other DNA
tcatgtttgaaatcctcaactctgacgg

SEQ ID NO: 25788 - DNA, 28 bp, synthetic construct
  source 1..28: mol_type = other DNA
tgatagcatttaccgcaaacgctgatgg

SEQ ID NO: 25789 - DNA, 28 bp, synthetic construct
  source 1..28: mol_type = other DNA
ggagagcaactgccatcagcgtttgcgg

SEQ ID NO: 25790 - DNA, 28 bp, synthetic construct
  source 1..28: mol_type = other DNA
tgctctcctttgccttatagctaactgg

SEQ ID NO: 25791 - DNA, 28 bp, synthetic construct
  source 1..28: mol_type = other DNA
gctctcctttgccttatagctaactggg

SEQ ID NO: 25792 - DNA, 28 bp, synthetic construct
  source 1..28: mol_type = other DNA
ctagtcccagttagctataaggcaaagg

SEQ ID NO: 25793 - DNA, 28 bp, synthetic construct
  source 1..28: mol_type = other DNA
ctgtttctagtcccagttagctataagg

SEQ ID NO: 25794 - DNA, 28 bp, synthetic construct
  source 1..28: mol_type = other DNA
gggactagaaacagctccatcacccagg

SEQ ID NO: 25795 - DNA, 28 bp, synthetic construct
  source 1..28: mol_type = other DNA
ctccatcacccaggtgagttttataagg

SEQ ID NO: 25796 - DNA, 28 bp, synthetic construct
  source 1..28: mol_type = other DNA
ttccttataaaactcacctgggtgatgg

SEQ ID NO: 25797 - DNA, 28 bp, synthetic construct
  source 1..28: mol_type = other DNA
ttatgtttccttataaaactcacctggg

SEQ ID NO: 25798 - DNA, 28 bp, synthetic construct
  source 1..28: mol_type = other DNA
cttatgtttccttataaaactcacctgg

SEQ ID NO: 25799 - DNA, 28 bp, synthetic construct
  source 1..28: mol_type = other DNA
caggtgagttttataaggaaacataagg

SEQ ID NO: 25800 - DNA, 28 bp, synthetic construct
  source 1..28: mol_type = other DNA
aggtgagttttataaggaaacataaggg

SEQ ID NO: 25801 - DNA, 28 bp, synthetic construct
  source 1..28: mol_type = other DNA
ggtgagttttataaggaaacataagggg

SEQ ID NO: 25802 - DNA, 28 bp, synthetic construct
  source 1..28: mol_type = other DNA
gtgagttttataaggaaacataaggggg

SEQ ID NO: 25803 - DNA, 28 bp, synthetic construct
  source 1..28: mol_type = other DNA
gttttataaggaaacataagggggctgg

SEQ ID NO: 25804 - DNA, 28 bp, synthetic construct
  source 1..28: mol_type = other DNA
gttgcttccctcctcttgtaagctttgg

SEQ ID NO: 25805 - DNA, 28 bp, synthetic construct
  source 1..28: mol_type = other DNA
gagttatccaaagcttacaagaggaggg

SEQ ID NO: 25806 - DNA, 28 bp, synthetic construct
  source 1..28: mol_type = other DNA
agagttatccaaagcttacaagaggagg

SEQ ID NO: 25807 - DNA, 28 bp, synthetic construct
  source 1..28: mol_type = other DNA
ttcagagttatccaaagcttacaagagg

SEQ ID NO: 25808 - DNA, 28 bp, synthetic construct
  source 1..28: mol_type = other DNA
agatatttctgaagatatttaaagaagg

SEQ ID NO: 25809 - DNA, 28 bp, synthetic construct
  source 1..28: mol_type = other DNA
atttctaagaagtttgaagattcagtgg

SEQ ID NO: 25810 - DNA, 28 bp, synthetic construct
  source 1..28: mol_type = other DNA
tttgaagattcagtggacacacttttgg

SEQ ID NO: 25811 - DNA, 28 bp, synthetic construct
  source 1..28: mol_type = other DNA
attgcattataaaagttttgattagtgg

SEQ ID NO: 25812 - DNA, 28 bp, synthetic construct
  source 1..28: mol_type = other DNA
gtaacaagtaaagagaaagaaaacatgg

SEQ ID NO: 25813 - DNA, 28 bp, synthetic construct
  source 1..28: mol_type = other DNA
agagaaagaaaacatggatctgcctagg

SEQ ID NO: 25814 - DNA, 28 bp, synthetic construct
  source 1..28: mol_type = other DNA
cagactcaggcagaggtgacttcctagg

SEQ ID NO: 25815 - DNA, 28 bp, synthetic construct
  source 1..28: mol_type = other DNA
acctctgcctgagtctgctacttgcagg

SEQ ID NO: 25816 - DNA, 28 bp, synthetic construct
  source 1..28: mol_type = other DNA
tcctgcaagtagcagactcaggcagagg

SEQ ID NO: 25817 - DNA, 28 bp, synthetic construct
  source 1..28: mol_type = other DNA
tgcctgagtctgctacttgcaggattgg

SEQ ID NO: 25818 - DNA, 28 bp, synthetic construct
  source 1..28: mol_type = other DNA
ctccaatcctgcaagtagcagactcagg

SEQ ID NO: 25819 - DNA, 28 bp, synthetic construct
  source 1..28: mol_type = other DNA
cacaataaaatataaactgctcttgagg

SEQ ID NO: 25820 - DNA, 28 bp, synthetic construct
  source 1..28: mol_type = other DNA
tgctttaaaaaaaaaatttagtgccagg

SEQ ID NO: 25821 - DNA, 28 bp, synthetic construct
  source 1..28: mol_type = other DNA
aaaaaaaaatttagtgccaggtttatgg

SEQ ID NO: 25822 - DNA, 28 bp, synthetic construct
  source 1..28: mol_type = other DNA
atgaaagcacttcactccataaacctgg

SEQ ID NO: 25823 - DNA, 28 bp, synthetic construct
  source 1..28: mol_type = other DNA
ataaatgctgaaactacattttctgtgg

SEQ ID NO: 25824 - DNA, 28 bp, synthetic construct
  source 1..28: mol_type = other DNA
taaatgctgaaactacattttctgtggg

SEQ ID NO: 25825 - DNA, 28 bp, synthetic construct
  source 1..28: mol_type = other DNA
tgtgaacataaaaaattcttcaaagggg

SEQ ID NO: 25826 - DNA, 28 bp, synthetic construct
  source 1..28: mol_type = other DNA
atgtgaacataaaaaattcttcaaaggg

SEQ ID NO: 25827 - DNA, 28 bp, synthetic construct
  source 1..28: mol_type = other DNA
tatgtgaacataaaaaattcttcaaagg

SEQ ID NO: 25828 - DNA, 28 bp, synthetic construct
  source 1..28: mol_type = other DNA
ctgtagggagatcaaatttttaacttgg

SEQ ID NO: 25829 - DNA, 28 bp, synthetic construct
  source 1..28: mol_type = other DNA
ttgaaatgaaagctcttactctgtaggg

SEQ ID NO: 25830 - DNA, 28 bp, synthetic construct
  source 1..28: mol_type = other DNA
tttgaaatgaaagctcttactctgtagg

SEQ ID NO: 25831 - DNA, 28 bp, synthetic construct
  source 1..28: mol_type = other DNA
ttcaaataaaaccattttatagaccagg

SEQ ID NO: 25832 - DNA, 28 bp, synthetic construct
  source 1..28: mol_type = other DNA
aaatgttgatacctggtctataaaatgg

SEQ ID NO: 25833 - DNA, 28 bp, synthetic construct
  source 1..28: mol_type = other DNA
tttatagaccaggtatcaacatttacgg

SEQ ID NO: 25834 - DNA, 28 bp, synthetic construct
  source 1..28: mol_type = other DNA
atagaccaggtatcaacatttacggcgg

SEQ ID NO: 25835 - DNA, 28 bp, synthetic construct
  source 1..28: mol_type = other DNA
atctcacacactctttcacatttctggg

SEQ ID NO: 25836 - DNA, 28 bp, synthetic construct
  source 1..28: mol_type = other DNA
catctcacacactctttcacatttctgg

SEQ ID NO: 25837 - DNA, 28 bp, synthetic construct
  source 1..28: mol_type = other DNA
cagaaatgtgaaagagtgtgtgagatgg

SEQ ID NO: 25838 - DNA, 28 bp, synthetic construct
  source 1..28: mol_type = other DNA
agaaatgtgaaagagtgtgtgagatggg

SEQ ID NO: 25839 - DNA, 28 bp, synthetic construct
  source 1..28: mol_type = other DNA
gggcttgcctctagagacttatctttgg

SEQ ID NO: 25840 - DNA, 28 bp, synthetic construct
  source 1..28: mol_type = other DNA
gaaagttccaaagataagtctctagagg

SEQ ID NO: 25841 - DNA, 28 bp, synthetic construct
  source 1..28: mol_type = other DNA
tctttggaactttcccagtgatctgtgg

SEQ ID NO: 25842 - DNA, 28 bp, synthetic construct
  source 1..28: mol_type = other DNA
atcacattgtggtccacagatcactggg

SEQ ID NO: 25843 - DNA, 28 bp, synthetic construct
  source 1..28: mol_type = other DNA
aatcacattgtggtccacagatcactgg

SEQ ID NO: 25844 - DNA, 28 bp, synthetic construct
  source 1..28: mol_type = other DNA
aaggggagggtgtgagcagaaaagcggg

SEQ ID NO: 25845 - DNA, 28 bp, synthetic construct
  source 1..28: mol_type = other DNA
gaaggggagggtgtgagcagaaaagcgg

SEQ ID NO: 25846 - DNA, 28 bp, synthetic construct
  source 1..28: mol_type = other DNA
taaaaaaatatagtgtggaaggggaggg

SEQ ID NO: 25847 - DNA, 28 bp, synthetic construct
  source 1..28: mol_type = other DNA
ttaaaaaaatatagtgtggaaggggagg

SEQ ID NO: 25848 - DNA, 28 bp, synthetic construct
  source 1..28: mol_type = other DNA
tttttaaaaaaatatagtgtggaagggg

SEQ ID NO: 25849 - DNA, 28 bp, synthetic construct
  source 1..28: mol_type = other DNA
ctttttaaaaaaatatagtgtggaaggg

SEQ ID NO: 25850 - DNA, 28 bp, synthetic construct
  source 1..28: mol_type = other DNA
tctttttaaaaaaatatagtgtggaagg

SEQ ID NO: 25851 - DNA, 28 bp, synthetic construct
  source 1..28: mol_type = other DNA
actgtctttttaaaaaaatatagtgtgg

SEQ ID NO: 25852 - DNA, 28 bp, synthetic construct
  source 1..28: mol_type = other DNA
acttcttgtaactacatgctaattctgg

SEQ ID NO: 25853 - DNA, 28 bp, synthetic construct
  source 1..28: mol_type = other DNA
ggagaaacaatgaaaggtcacaactagg

SEQ ID NO: 25854 - DNA, 28 bp, synthetic construct
  source 1..28: mol_type = other DNA
aaaatgggaaaggagaaacaatgaaagg

SEQ ID NO: 25855 - DNA, 28 bp, synthetic construct
  source 1..28: mol_type = other DNA
tcataaaacaaatgaaaaatgggaaagg

SEQ ID NO: 25856 - DNA, 28 bp, synthetic construct
  source 1..28: mol_type = other DNA
cttagtcataaaacaaatgaaaaatggg

SEQ ID NO: 25857 - DNA, 28 bp, synthetic construct
  source 1..28: mol_type = other DNA
acttagtcataaaacaaatgaaaaatgg

SEQ ID NO: 25858 - DNA, 28 bp, synthetic construct
  source 1..28: mol_type = other DNA
tttcatttgttttatgactaagtaatgg

SEQ ID NO: 25859 - DNA, 28 bp, synthetic construct
  source 1..28: mol_type = other DNA
tggcacttaaataaaataatacagtagg

SEQ ID NO: 25860 - DNA, 28 bp, synthetic construct
  source 1..28: mol_type = other DNA
cacttaaataaaataatacagtaggagg

SEQ ID NO: 25861 - DNA, 28 bp, synthetic construct
  source 1..28: mol_type = other DNA
aaaataatacagtaggaggcagcaaagg

SEQ ID NO: 25862 - DNA, 28 bp, synthetic construct
  source 1..28: mol_type = other DNA
acagactttaaaacaatgctaaaaaagg

SEQ ID NO: 25863 - DNA, 28 bp, synthetic construct
  source 1..28: mol_type = other DNA
cagactttaaaacaatgctaaaaaaggg

SEQ ID NO: 25864 - DNA, 28 bp, synthetic construct
  source 1..28: mol_type = other DNA
gatagtctagaaatactattaacatagg

SEQ ID NO: 25865 - DNA, 28 bp, synthetic construct
  source 1..28: mol_type = other DNA
aaggggagtacagaaacacactacatgg

SEQ ID NO: 25866 - DNA, 28 bp, synthetic construct
  source 1..28: mol_type = other DNA
tttctgtactccccttgtgcattttagg

SEQ ID NO: 25867 - DNA, 28 bp, synthetic construct
  source 1..28: mol_type = other DNA
ttaactttgacctaaaatgcacaagggg

SEQ ID NO: 25868 - DNA, 28 bp, synthetic construct
  source 1..28: mol_type = other DNA
tttaactttgacctaaaatgcacaaggg

SEQ ID NO: 25869 - DNA, 28 bp, synthetic construct
  source 1..28: mol_type = other DNA
ctttaactttgacctaaaatgcacaagg

SEQ ID NO: 25870 - DNA, 28 bp, synthetic construct
  source 1..28: mol_type = other DNA
cttgtgcattttaggtcaaagttaaagg

SEQ ID NO: 25871 - DNA, 28 bp, synthetic construct
  source 1..28: mol_type = other DNA
acaacatcttttgtcacttagcgcatgg

SEQ ID NO: 25872 - DNA, 28 bp, synthetic construct
  source 1..28: mol_type = other DNA
caacatcttttgtcacttagcgcatggg

SEQ ID NO: 25873 - DNA, 28 bp, synthetic construct
  source 1..28: mol_type = other DNA
gcaggagagtcttttacatgagtgctgg

SEQ ID NO: 25874 - DNA, 28 bp, synthetic construct
  source 1..28: mol_type = other DNA
tgtaaaagactctcctgcaatttgcagg

SEQ ID NO: 25875 - DNA, 28 bp, synthetic construct
  source 1..28: mol_type = other DNA
gtaaaagactctcctgcaatttgcaggg

SEQ ID NO: 25876 - DNA, 28 bp, synthetic construct
  source 1..28: mol_type = other DNA
aaagactctcctgcaatttgcagggtgg

SEQ ID NO: 25877 - DNA, 28 bp, synthetic construct
  source 1..28: mol_type = other DNA
ctcctgcaatttgcagggtggcccgagg

SEQ ID NO: 25878 - DNA, 28 bp, synthetic construct
  source 1..28: mol_type = other DNA
ttcctcgggccaccctgcaaattgcagg

SEQ ID NO: 25879 - DNA, 28 bp, synthetic construct
  source 1..28: mol_type = other DNA
aatttgcagggtggcccgaggaagcagg

SEQ ID NO: 25880 - DNA, 28 bp, synthetic construct
  source 1..28: mol_type = other DNA
atttgcagggtggcccgaggaagcaggg

SEQ ID NO: 25881 - DNA, 28 bp, synthetic construct
  source 1..28: mol_type = other DNA
aagggcaatggctccctgcttcctcggg

SEQ ID NO: 25882 - DNA, 28 bp, synthetic construct
  source 1..28: mol_type = other DNA
caagggcaatggctccctgcttcctcgg

SEQ ID NO: 25883 - DNA, 28 bp, synthetic construct
  source 1..28: mol_type = other DNA
acagcaatgggctctgcaagggcaatgg

SEQ ID NO: 25884 - DNA, 28 bp, synthetic construct
  source 1..28: mol_type = other DNA
cccttgcagagcccattgctgtctttgg

SEQ ID NO: 25885 - DNA, 28 bp, synthetic construct
  source 1..28: mol_type = other DNA
tccaaagacagcaatgggctctgcaagg

SEQ ID NO: 25886 - DNA, 28 bp, synthetic construct
  source 1..28: mol_type = other DNA
caattaaatgtccaaagacagcaatggg

SEQ ID NO: 25887 - DNA, 28 bp, synthetic construct
  source 1..28: mol_type = other DNA
acaattaaatgtccaaagacagcaatgg

SEQ ID NO: 25888 - DNA, 28 bp, synthetic construct
  source 1..28: mol_type = other DNA
ggacatttaattgttgaaatgtattagg

SEQ ID NO: 25889 - DNA, 28 bp, synthetic construct
  source 1..28: mol_type = other DNA
catttaattgttgaaatgtattaggagg

SEQ ID NO: 25890 - DNA, 28 bp, synthetic construct
  source 1..28: mol_type = other DNA
ggccgctaatcaatagcctgtaatttgg

SEQ ID NO: 25891 - DNA, 28 bp, synthetic construct
  source 1..28: mol_type = other DNA
gccgctaatcaatagcctgtaatttggg

SEQ ID NO: 25892 - DNA, 28 bp, synthetic construct
  source 1..28: mol_type = other DNA
gcccaaattacaggctattgattagcgg

SEQ ID NO: 25893 - DNA, 28 bp, synthetic construct
  source 1..28: mol_type = other DNA
ataaagtttttacagcccaaattacagg

SEQ ID NO: 25894 - DNA, 28 bp, synthetic construct
  source 1..28: mol_type = other DNA
aatcaagaacatagctcaaaataagtgg

SEQ ID NO: 25895 - DNA, 28 bp, synthetic construct
  source 1..28: mol_type = other DNA
ttctactaactacagaagatgacatagg

SEQ ID NO: 25896 - DNA, 28 bp, synthetic construct
  source 1..28: mol_type = other DNA
tgtcatcttctgtagttagtagaagcgg

SEQ ID NO: 25897 - DNA, 28 bp, synthetic construct
  source 1..28: mol_type = other DNA
agcggtgttttttgtttgttttacctgg

SEQ ID NO: 25898 - DNA, 28 bp, synthetic construct
  source 1..28: mol_type = other DNA
gcggtgttttttgtttgttttacctggg

SEQ ID NO: 25899 - DNA, 28 bp, synthetic construct
  source 1..28: mol_type = other DNA
cggtgttttttgtttgttttacctgggg

SEQ ID NO: 25900 - DNA, 28 bp, synthetic construct
  source 1..28: mol_type = other DNA
ggtgttttttgtttgttttacctggggg

SEQ ID NO: 25901 - DNA, 28 bp, synthetic construct
  source 1..28: mol_type = other DNA
tgtttgttttacctgggggcaatgtagg

SEQ ID NO: 25902 - DNA, 28 bp, synthetic construct
  source 1..28: mol_type = other DNA
cctgggggcaatgtaggtgaccatttgg

SEQ ID NO: 25903 - DNA, 28 bp, synthetic construct
  source 1..28: mol_type = other DNA
tgaccatttggacacctttttcacatgg

SEQ ID NO: 25904 - DNA, 28 bp, synthetic construct
  source 1..28: mol_type = other DNA
gaccatttggacacctttttcacatggg

SEQ ID NO: 25905 - DNA, 28 bp, synthetic construct
  source 1..28: mol_type = other DNA
gtcccatgtgaaaaaggtgtccaaatgg

SEQ ID NO: 25906 - DNA, 28 bp, synthetic construct
  source 1..28: mol_type = other DNA
caaacaaaagtgtcccatgtgaaaaagg

SEQ ID NO: 25907 - DNA, 28 bp, synthetic construct
  source 1..28: mol_type = other DNA
tttgtgtgtgtgtttgtttttgagacgg

SEQ ID NO: 25908 - DNA, 28 bp, synthetic construct
  source 1..28: mol_type = other DNA
tgagacggagtcttgctctgtcaccagg

SEQ ID NO: 25909 - DNA, 28 bp, synthetic construct
  source 1..28: mol_type = other DNA
gctctgtcaccaggctgaagtgcagtgg

SEQ ID NO: 25910 - DNA, 28 bp, synthetic construct
  source 1..28: mol_type = other DNA
gggattgcgccactgcacttcagcctgg

SEQ ID NO: 25911 - DNA, 28 bp, synthetic construct
  source 1..28: mol_type = other DNA
tgggaggcggaggttgcagtgagctggg

SEQ ID NO: 25912 - DNA, 28 bp, synthetic construct
  source 1..28: mol_type = other DNA
ctgggaggcggaggttgcagtgagctgg

SEQ ID NO: 25913 - DNA, 28 bp, synthetic construct
  source 1..28: mol_type = other DNA
cagctcactgcaacctccgcctcccagg

SEQ ID NO: 25914 - DNA, 28 bp, synthetic construct
  source 1..28: mol_type = other DNA
agaatcacttgaacctgggaggcggagg

SEQ ID NO: 25915 - DNA, 28 bp, synthetic construct
  source 1..28: mol_type = other DNA
aggagaatcacttgaacctgggaggcgg

SEQ ID NO: 25916 - DNA, 28 bp, synthetic construct
  source 1..28: mol_type = other DNA
ggcaggagaatcacttgaacctgggagg

SEQ ID NO: 25917 - DNA, 28 bp, synthetic construct
  source 1..28: mol_type = other DNA
tgaggcaggagaatcacttgaacctggg

SEQ ID NO: 25918 - DNA, 28 bp, synthetic construct
  source 1..28: mol_type = other DNA
ctgaggcaggagaatcacttgaacctgg

SEQ ID NO: 25919 - DNA, 28 bp, synthetic construct
  source 1..28: mol_type = other DNA
ctcctgcctcagcctcttgagtagctgg

SEQ ID NO: 25920 - DNA, 28 bp, synthetic construct
  source 1..28: mol_type = other DNA
tcctgcctcagcctcttgagtagctggg

SEQ ID NO: 25921 - DNA, 28 bp, synthetic construct
  source 1..28: mol_type = other DNA
tcccagctactcaagaggctgaggcagg

SEQ ID NO: 25922 - DNA, 28 bp, synthetic construct
  source 1..28: mol_type = other DNA
gtaatcccagctactcaagaggctgagg

SEQ ID NO: 25923 - DNA, 28 bp, synthetic construct
  source 1..28: mol_type = other DNA
cagcctcttgagtagctgggattacagg

SEQ ID NO: 25924 - DNA, 28 bp, synthetic construct
  source 1..28: mol_type = other DNA
gcgcctgtaatcccagctactcaagagg

SEQ ID NO: 25925 - DNA, 28 bp, synthetic construct
  source 1..28: mol_type = other DNA
tacaaaactagctgggtgtggttgcagg

SEQ ID NO: 25926 - DNA, 28 bp, synthetic construct
  source 1..28: mol_type = other DNA
ctaaaaatacaaaactagctgggtgtgg

SEQ ID NO: 25927 - DNA, 28 bp, synthetic construct
  source 1..28: mol_type = other DNA
ctcaactaaaaatacaaaactagctggg

SEQ ID NO: 25928 - DNA, 28 bp, synthetic construct
  source 1..28: mol_type = other DNA
tctcaactaaaaatacaaaactagctgg

SEQ ID NO: 25929 - DNA, 28 bp, synthetic construct
  source 1..28: mol_type = other DNA
gctagttttgtatttttagttgagatgg

SEQ ID NO: 25930 - DNA, 28 bp, synthetic construct
  source 1..28: mol_type = other DNA
ctagttttgtatttttagttgagatggg

SEQ ID NO: 25931 - DNA, 28 bp, synthetic construct
  source 1..28: mol_type = other DNA
tagttttgtatttttagttgagatgggg

SEQ ID NO: 25932 - DNA, 28 bp, synthetic construct
  source 1..28: mol_type = other DNA
gagatggggtttcaccatattgtccagg

SEQ ID NO: 25933 - DNA, 28 bp, synthetic construct
  source 1..28: mol_type = other DNA
gaaatcgagatcatcctggacaatatgg

SEQ ID NO: 25934 - DNA, 28 bp, synthetic construct
  source 1..28: mol_type = other DNA
cagagtcaggaaatcgagatcatcctgg

SEQ ID NO: 25935 - DNA, 28 bp, synthetic construct
  source 1..28: mol_type = other DNA
tcctgactctgtgatctgcctgcctcgg

SEQ ID NO: 25936 - DNA, 28 bp, synthetic construct
  source 1..28: mol_type = other DNA
gccgaggcaggcagatcacagagtcagg

SEQ ID NO: 25937 - DNA, 28 bp, synthetic construct
  source 1..28: mol_type = other DNA
tgcctgcctcggcctcccaaagtgctgg

SEQ ID NO: 25938 - DNA, 28 bp, synthetic construct
  source 1..28: mol_type = other DNA
gcctgcctcggcctcccaaagtgctggg

SEQ ID NO: 25939 - DNA, 28 bp, synthetic construct
  source 1..28: mol_type = other DNA
tcccagcactttgggaggccgaggcagg

SEQ ID NO: 25940 - DNA, 28 bp, synthetic construct
  source 1..28: mol_type = other DNA
gtaatcccagcactttgggaggccgagg

SEQ ID NO: 25941 - DNA, 28 bp, synthetic construct
  source 1..28: mol_type = other DNA
cggcctcccaaagtgctgggattacagg

SEQ ID NO: 25942 - DNA, 28 bp, synthetic construct
  source 1..28: mol_type = other DNA
acacctgtaatcccagcactttgggagg

SEQ ID NO: 25943 - DNA, 28 bp, synthetic construct
  source 1..28: mol_type = other DNA
ctcacacctgtaatcccagcactttggg

SEQ ID NO: 25944 - DNA, 28 bp, synthetic construct
  source 1..28: mol_type = other DNA
gctcacacctgtaatcccagcactttgg

SEQ ID NO: 25945 - DNA, 28 bp, synthetic construct
  source 1..28: mol_type = other DNA
gattacaggtgtgagcctctgcgcctgg

SEQ ID NO: 25946 - DNA, 28 bp, synthetic construct
  source 1..28: mol_type = other DNA
gtgtgagcctctgcgcctggccgcatgg

SEQ ID NO: 25947 - DNA, 28 bp, synthetic construct
  source 1..28: mol_type = other DNA
tgtgagcctctgcgcctggccgcatggg

SEQ ID NO: 25948 - DNA, 28 bp, synthetic construct
  source 1..28: mol_type = other DNA
atgtctcccatgcggccaggcgcagagg

SEQ ID NO: 25949 - DNA, 28 bp, synthetic construct
  source 1..28: mol_type = other DNA
atttaaaaatgtctcccatgcggccagg

SEQ ID NO: 25950 - DNA, 28 bp, synthetic construct
  source 1..28: mol_type = other DNA
tacacatttaaaaatgtctcccatgcgg

SEQ ID NO: 25951 - DNA, 28 bp, synthetic construct
  source 1..28: mol_type = other DNA
ttttaaatgtgtagactttgactccagg

SEQ ID NO: 25952 - DNA, 28 bp, synthetic construct
  source 1..28: mol_type = other DNA
ctttgactccaggagttagtaccattgg

SEQ ID NO: 25953 - DNA, 28 bp, synthetic construct
  source 1..28: mol_type = other DNA
tttgactccaggagttagtaccattggg

SEQ ID NO: 25954 - DNA, 28 bp, synthetic construct
  source 1..28: mol_type = other DNA
aggtgttcccaatggtactaactcctgg

SEQ ID NO: 25955 - DNA, 28 bp, synthetic construct
  source 1..28: mol_type = other DNA
cggaagcagtcacaggtgttcccaatgg

SEQ ID NO: 25956 - DNA, 28 bp, synthetic construct
  source 1..28: mol_type = other DNA
gaacacctgtgactgcttccgctaaagg

SEQ ID NO: 25957 - DNA, 28 bp, synthetic construct
  source 1..28: mol_type = other DNA
aacacctgtgactgcttccgctaaaggg

SEQ ID NO: 25958 - DNA, 28 bp, synthetic construct
  source 1..28: mol_type = other DNA
tgtaccctttagcggaagcagtcacagg

SEQ ID NO: 25959 - DNA, 28 bp, synthetic construct
  source 1..28: mol_type = other DNA
acacatttgctagtgtaccctttagcgg

SEQ ID NO: 25960 - DNA, 28 bp, synthetic construct
  source 1..28: mol_type = other DNA
acagagttttaaacacctcatataaagg

SEQ ID NO: 25961 - DNA, 28 bp, synthetic construct
  source 1..28: mol_type = other DNA
tcaactgaattaatacctttatatgagg

SEQ ID NO: 25962 - DNA, 28 bp, synthetic construct
  source 1..28: mol_type = other DNA
tattaattcagttgatttatccaaaagg

SEQ ID NO: 25963 - DNA, 28 bp, synthetic construct
  source 1..28: mol_type = other DNA
aaaataagaattagtgtcttccttttgg

SEQ ID NO: 25964 - DNA, 28 bp, synthetic construct
  source 1..28: mol_type = other DNA
aaggaagacactaattcttattttgtgg

SEQ ID NO: 25965 - DNA, 28 bp, synthetic construct
  source 1..28: mol_type = other DNA
agaaaaaaaagagctaaaagagaagggg

SEQ ID NO: 25966 - DNA, 28 bp, synthetic construct
  source 1..28: mol_type = other DNA
cagaaaaaaaagagctaaaagagaaggg

SEQ ID NO: 25967 - DNA, 28 bp, synthetic construct
  source 1..28: mol_type = other DNA
tcagaaaaaaaagagctaaaagagaagg

SEQ ID NO: 25968 - DNA, 28 bp, synthetic construct
  source 1..28: mol_type = other DNA
aacagattaaaaaaaaacttttaagagg

SEQ ID NO: 25969 - DNA, 28 bp, synthetic construct
  source 1..28: mol_type = other DNA
aaagtttttttttaatctgttttctagg

SEQ ID NO: 25970 - DNA, 28 bp, synthetic construct
  source 1..28: mol_type = other DNA
aagtttttttttaatctgttttctaggg

SEQ ID NO: 25971 - DNA, 28 bp, synthetic construct
  source 1..28: mol_type = other DNA
agtttttttttaatctgttttctagggg

SEQ ID NO: 25972 - DNA, 28 bp, synthetic construct
  source 1..28: mol_type = other DNA
ttttttttaatctgttttctaggggagg

SEQ ID NO: 25973 - DNA, 28 bp, synthetic construct
  source 1..28: mol_type = other DNA
tctgttttctaggggaggtcatgcttgg

SEQ ID NO: 25974 - DNA, 28 bp, synthetic construct
  source 1..28: mol_type = other DNA
gcttggttaattgttgctaagtaaatgg

SEQ ID NO: 25975 - DNA, 28 bp, synthetic construct
  source 1..28: mol_type = other DNA
ataaaggcagaaaaataataatcaaagg

SEQ ID NO: 25976 - DNA, 28 bp, synthetic construct
  source 1..28: mol_type = other DNA
tttctgcctttatacaatgtgttttagg

SEQ ID NO: 25977 - DNA, 28 bp, synthetic construct
  source 1..28: mol_type = other DNA
aagaagcctaaaacacattgtataaagg

SEQ ID NO: 25978 - DNA, 28 bp, synthetic construct
  source 1..28: mol_type = other DNA
acaaatagacattttcccattacaaagg

SEQ ID NO: 25979 - DNA, 28 bp, synthetic construct
  source 1..28: mol_type = other DNA
aagaactgatagtgtcctttgtaatggg

SEQ ID NO: 25980 - DNA, 28 bp, synthetic construct
  source 1..28: mol_type = other DNA
gaagaactgatagtgtcctttgtaatgg

SEQ ID NO: 25981 - DNA, 28 bp, synthetic construct
  source 1..28: mol_type = other DNA
aaaggacactatcagttcttcagtatgg

SEQ ID NO: 25982 - DNA, 28 bp, synthetic construct
  source 1..28: mol_type = other DNA
ctgtaagagtcaagaaaacacacatcgg

SEQ ID NO: 25983 - DNA, 28 bp, synthetic construct
  source 1..28: mol_type = other DNA
cacatcggatcttcctacctttctgtgg

SEQ ID NO: 25984 - DNA, 28 bp, synthetic construct
  source 1..28: mol_type = other DNA
acatcggatcttcctacctttctgtggg

SEQ ID NO: 25985 - DNA, 28 bp, synthetic construct
  source 1..28: mol_type = other DNA
catcggatcttcctacctttctgtgggg

SEQ ID NO: 25986 - DNA, 28 bp, synthetic construct
  source 1..28: mol_type = other DNA
atcggatcttcctacctttctgtggggg

SEQ ID NO: 25987 - DNA, 28 bp, synthetic construct
  source 1..28: mol_type = other DNA
tcctacctttctgtgggggtgtttgagg

SEQ ID NO: 25988 - DNA, 28 bp, synthetic construct
  source 1..28: mol_type = other DNA
tcctcaaacacccccacagaaaggtagg

SEQ ID NO: 25989 - DNA, 28 bp, synthetic construct
  source 1..28: mol_type = other DNA
actctcctcaaacacccccacagaaagg

SEQ ID NO: 25990 - DNA, 28 bp, synthetic construct
  source 1..28: mol_type = other DNA
ctgtagtaatgattctgttgtaaaatgg

SEQ ID NO: 25991 - DNA, 28 bp, synthetic construct
  source 1..28: mol_type = other DNA
tgtagtaatgattctgttgtaaaatggg

SEQ ID NO: 25992 - DNA, 28 bp, synthetic construct
  source 1..28: mol_type = other DNA
tgtaaaatgggaagtgtgacattgatgg

SEQ ID NO: 25993 - DNA, 28 bp, synthetic construct
  source 1..28: mol_type = other DNA
aatttcttaaaatactgtcttaagctgg

SEQ ID NO: 25994 - DNA, 28 bp, synthetic construct
  source 1..28: mol_type = other DNA
tactgtcttaagctggcaaaactcctgg

SEQ ID NO: 25995 - DNA, 28 bp, synthetic construct
  source 1..28: mol_type = other DNA
tggtttatgtcaggtggaggatgccagg

SEQ ID NO: 25996 - DNA, 28 bp, synthetic construct
  source 1..28: mol_type = other DNA
ctgtgaactggtttatgtcaggtggagg

SEQ ID NO: 25997 - DNA, 28 bp, synthetic construct
  source 1..28: mol_type = other DNA
gttctgtgaactggtttatgtcaggtgg

SEQ ID NO: 25998 - DNA, 28 bp, synthetic construct
  source 1..28: mol_type = other DNA
aatgttctgtgaactggtttatgtcagg

SEQ ID NO: 25999 - DNA, 28 bp, synthetic construct
  source 1..28: mol_type = other DNA
atctaggctggaatgttctgtgaactgg

SEQ ID NO: 26000 - DNA, 28 bp, synthetic construct
  source 1..28: mol_type = other DNA
agaacattccagcctagatctgaaatgg

SEQ ID NO: 26001 - DNA, 28 bp, synthetic construct
  source 1..28: mol_type = other DNA
aaaaattaccatttcagatctaggctgg

SEQ ID NO: 26002 - DNA, 28 bp, synthetic construct
  source 1..28: mol_type = other DNA
cctagatctgaaatggtaatttttttgg

SEQ ID NO: 26003 - DNA, 28 bp, synthetic construct
  source 1..28: mol_type = other DNA
tgaaatggtaatttttttggaactttgg

SEQ ID NO: 26004 - DNA, 28 bp, synthetic construct
  source 1..28: mol_type = other DNA
atggtaatttttttggaactttggttgg

SEQ ID NO: 26005 - DNA, 28 bp, synthetic construct
  source 1..28: mol_type = other DNA
accattccctccagttcctctgccttgg

SEQ ID NO: 26006 - DNA, 28 bp, synthetic construct
  source 1..28: mol_type = other DNA
accaaggcagaggaactggagggaatgg

SEQ ID NO: 26007 - DNA, 28 bp, synthetic construct
  source 1..28: mol_type = other DNA
ggtaaaccaaggcagaggaactggaggg

SEQ ID NO: 26008 - DNA, 28 bp, synthetic construct
  source 1..28: mol_type = other DNA
aggtaaaccaaggcagaggaactggagg

SEQ ID NO: 26009 - DNA, 28 bp, synthetic construct
  source 1..28: mol_type = other DNA
tttaggtaaaccaaggcagaggaactgg

SEQ ID NO: 26010 - DNA, 28 bp, synthetic construct
  source 1..28: mol_type = other DNA
agttcctctgccttggtttacctaaagg

SEQ ID NO: 26011 - DNA, 28 bp, synthetic construct
  source 1..28: mol_type = other DNA
gttcctctgccttggtttacctaaaggg

SEQ ID NO: 26012 - DNA, 28 bp, synthetic construct
  source 1..28: mol_type = other DNA
aatccctttaggtaaaccaaggcagagg

SEQ ID NO: 26013 - DNA, 28 bp, synthetic construct
  source 1..28: mol_type = other DNA
tgccttggtttacctaaagggattttgg

SEQ ID NO: 26014 - DNA, 28 bp, synthetic construct
  source 1..28: mol_type = other DNA
caccaaaatccctttaggtaaaccaagg

SEQ ID NO: 26015 - DNA, 28 bp, synthetic construct
  source 1..28: mol_type = other DNA
cacacaggaacaccaaaatccctttagg

SEQ ID NO: 26016 - DNA, 28 bp, synthetic construct
  source 1..28: mol_type = other DNA
ggattttggtgttcctgtgtgtgactgg

SEQ ID NO: 26017 - DNA, 28 bp, synthetic construct
  source 1..28: mol_type = other DNA
tggtgttcctgtgtgtgactggaagtgg

SEQ ID NO: 26018 - DNA, 28 bp, synthetic construct
  source 1..28: mol_type = other DNA
gagacagccacttccagtcacacacagg

SEQ ID NO: 26019 - DNA, 28 bp, synthetic construct
  source 1..28: mol_type = other DNA
ctggaagtggctgtctctattgactagg

SEQ ID NO: 26020 - DNA, 28 bp, synthetic construct
  source 1..28: mol_type = other DNA
gctgtctctattgactaggaagaactgg

SEQ ID NO: 26021 - DNA, 28 bp, synthetic construct
  source 1..28: mol_type = other DNA
ttgactaggaagaactggtgagaagtgg

SEQ ID NO: 26022 - DNA, 28 bp, synthetic construct
  source 1..28: mol_type = other DNA
tgactaggaagaactggtgagaagtggg

SEQ ID NO: 26023 - DNA, 28 bp, synthetic construct
  source 1..28: mol_type = other DNA
tgagaagtgggaccacagtgtattcagg

SEQ ID NO: 26024 - DNA, 28 bp, synthetic construct
  source 1..28: mol_type = other DNA
gaccacagtgtattcaggatcaaagtgg

SEQ ID NO: 26025 - DNA, 28 bp, synthetic construct
  source 1..28: mol_type = other DNA
accacagtgtattcaggatcaaagtggg

SEQ ID NO: 26026 - DNA, 28 bp, synthetic construct
  source 1..28: mol_type = other DNA
ccccactttgatcctgaatacactgtgg

SEQ ID NO: 26027 - DNA, 28 bp, synthetic construct
  source 1..28: mol_type = other DNA
cagtgtattcaggatcaaagtggggagg

SEQ ID NO: 26028 - DNA, 28 bp, synthetic construct
  source 1..28: mol_type = other DNA
tggggaggacatgagtccctttaagagg

SEQ ID NO: 26029 - DNA, 28 bp, synthetic construct
  source 1..28: mol_type = other DNA
ggggaggacatgagtccctttaagaggg

SEQ ID NO: 26030 - DNA, 28 bp, synthetic construct
  source 1..28: mol_type = other DNA
aggacatgagtccctttaagagggtagg

SEQ ID NO: 26031 - DNA, 28 bp, synthetic construct
  source 1..28: mol_type = other DNA
gagtgtattcacctaccctcttaaaggg

SEQ ID NO: 26032 - DNA, 28 bp, synthetic construct
  source 1..28: mol_type = other DNA
tgagtgtattcacctaccctcttaaagg

SEQ ID NO: 26033 - DNA, 28 bp, synthetic construct
  source 1..28: mol_type = other DNA
ggtgaatacactcaagtcccgattctgg

SEQ ID NO: 26034 - DNA, 28 bp, synthetic construct
  source 1..28: mol_type = other DNA
ggattctggacacaataccagaatcggg

SEQ ID NO: 26035 - DNA, 28 bp, synthetic construct
  source 1..28: mol_type = other DNA
tggattctggacacaataccagaatcgg

SEQ ID NO: 26036 - DNA, 28 bp, synthetic construct
  source 1..28: mol_type = other DNA
tctggtattgtgtccagaatccaacagg

SEQ ID NO: 26037 - DNA, 28 bp, synthetic construct
  source 1..28: mol_type = other DNA
agaaatgatctgtcctgttggattctgg

SEQ ID NO: 26038 - DNA, 28 bp, synthetic construct
  source 1..28: mol_type = other DNA
atccaacaggacagatcatttctgatgg

SEQ ID NO: 26039 - DNA, 28 bp, synthetic construct
  source 1..28: mol_type = other DNA
tccaacaggacagatcatttctgatggg

SEQ ID NO: 26040 - DNA, 28 bp, synthetic construct
  source 1..28: mol_type = other DNA
acccatcagaaatgatctgtcctgttgg

SEQ ID NO: 26041 - DNA, 28 bp, synthetic construct
  source 1..28: mol_type = other DNA
caggacagatcatttctgatgggtatgg

SEQ ID NO: 26042 - DNA, 28 bp, synthetic construct
  source 1..28: mol_type = other DNA
tgggtatggagacatctctgaacctagg

SEQ ID NO: 26043 - DNA, 28 bp, synthetic construct
  source 1..28: mol_type = other DNA
ccaggggatggtcagttcattgcctagg

SEQ ID NO: 26044 - DNA, 28 bp, synthetic construct
  source 1..28: mol_type = other DNA
ctaggcaatgaactgaccatcccctggg

SEQ ID NO: 26045 - DNA, 28 bp, synthetic construct
  source 1..28: mol_type = other DNA
acgggaaggagacaggcccaggggatgg

SEQ ID NO: 26046 - DNA, 28 bp, synthetic construct
  source 1..28: mol_type = other DNA
cccctgggcctgtctccttcccgtctgg

SEQ ID NO: 26047 - DNA, 28 bp, synthetic construct
  source 1..28: mol_type = other DNA
tccagacgggaaggagacaggcccaggg

SEQ ID NO: 26048 - DNA, 28 bp, synthetic construct
  source 1..28: mol_type = other DNA
ttccagacgggaaggagacaggcccagg

SEQ ID NO: 26049 - DNA, 28 bp, synthetic construct
  source 1..28: mol_type = other DNA
tgggcctgtctccttcccgtctggaagg

SEQ ID NO: 26050 - DNA, 28 bp, synthetic construct
  source 1..28: mol_type = other DNA
gggcctgtctccttcccgtctggaaggg

SEQ ID NO: 26051 - DNA, 28 bp, synthetic construct
  source 1..28: mol_type = other DNA
ggcctgtctccttcccgtctggaagggg

SEQ ID NO: 26052 - DNA, 28 bp, synthetic construct
  source 1..28: mol_type = other DNA
agccccttccagacgggaaggagacagg

SEQ ID NO: 26053 - DNA, 28 bp, synthetic construct
  source 1..28: mol_type = other DNA
tctacaaagccccttccagacgggaagg

SEQ ID NO: 26054 - DNA, 28 bp, synthetic construct
  source 1..28: mol_type = other DNA
ggtgtctacaaagccccttccagacggg

SEQ ID NO: 26055 - DNA, 28 bp, synthetic construct
  source 1..28: mol_type = other DNA
gggtgtctacaaagccccttccagacgg

SEQ ID NO: 26056 - DNA, 28 bp, synthetic construct
  source 1..28: mol_type = other DNA
ctggaaggggctttgtagacaccctcgg

SEQ ID NO: 26057 - DNA, 28 bp, synthetic construct
  source 1..28: mol_type = other DNA
tggaaggggctttgtagacaccctcggg

SEQ ID NO: 26058 - DNA, 28 bp, synthetic construct
  source 1..28: mol_type = other DNA
ggaaggggctttgtagacaccctcgggg

SEQ ID NO: 26059 - DNA, 28 bp, synthetic construct
  source 1..28: mol_type = other DNA
ccatctaaggcagatcttgccccgaggg

SEQ ID NO: 26060 - DNA, 28 bp, synthetic construct
  source 1..28: mol_type = other DNA
cctcggggcaagatctgccttagatggg

SEQ ID NO: 26061 - DNA, 28 bp, synthetic construct
  source 1..28: mol_type = other DNA
ctcggggcaagatctgccttagatgggg

SEQ ID NO: 26062 - DNA, 28 bp, synthetic construct
  source 1..28: mol_type = other DNA
tctttctctcaggcagccccatctaagg

SEQ ID NO: 26063 - DNA, 28 bp, synthetic construct
  source 1..28: mol_type = other DNA
ttagatggggctgcctgagagaaagagg

SEQ ID NO: 26064 - DNA, 28 bp, synthetic construct
  source 1..28: mol_type = other DNA
gatggggctgcctgagagaaagaggtgg

SEQ ID NO: 26065 - DNA, 28 bp, synthetic construct
  source 1..28: mol_type = other DNA
ctgcctgagagaaagaggtggcagtagg

SEQ ID NO: 26066 - DNA, 28 bp, synthetic construct
  source 1..28: mol_type = other DNA
aggcctactgccacctctttctctcagg

SEQ ID NO: 26067 - DNA, 28 bp, synthetic construct
  source 1..28: mol_type = other DNA
gaaagaggtggcagtaggccttgcctgg

SEQ ID NO: 26068 - DNA, 28 bp, synthetic construct
  source 1..28: mol_type = other DNA
agggagacactgtgggcaccaggcaagg

SEQ ID NO: 26069 - DNA, 28 bp, synthetic construct
  source 1..28: mol_type = other DNA
gcagcagggagacactgtgggcaccagg

SEQ ID NO: 26070 - DNA, 28 bp, synthetic construct
  source 1..28: mol_type = other DNA
gctcttggcagcagggagacactgtggg

SEQ ID NO: 26071 - DNA, 28 bp, synthetic construct
  source 1..28: mol_type = other DNA
agctcttggcagcagggagacactgtgg

SEQ ID NO: 26072 - DNA, 28 bp, synthetic construct
  source 1..28: mol_type = other DNA
agtgtctccctgctgccaagagctctgg

SEQ ID NO: 26073 - DNA, 28 bp, synthetic construct
  source 1..28: mol_type = other DNA
gtgtctccctgctgccaagagctctggg

SEQ ID NO: 26074 - DNA, 28 bp, synthetic construct
  source 1..28: mol_type = other DNA
tcagtacccagagctcttggcagcaggg

SEQ ID NO: 26075 - DNA, 28 bp, synthetic construct
  source 1..28: mol_type = other DNA
ctcagtacccagagctcttggcagcagg

SEQ ID NO: 26076 - DNA, 28 bp, synthetic construct
  source 1..28: mol_type = other DNA
agcttatctcagtacccagagctcttgg

SEQ ID NO: 26077 - DNA, 28 bp, synthetic construct
  source 1..28: mol_type = other DNA
actgagataagcttgcacattctcaagg

SEQ ID NO: 26078 - DNA, 28 bp, synthetic construct
  source 1..28: mol_type = other DNA
ctgttagagattttgaccgcagagctgg

SEQ ID NO: 26079 - DNA, 28 bp, synthetic construct
  source 1..28: mol_type = other DNA
ttgaccgcagagctggttgtgttaaagg

SEQ ID NO: 26080 - DNA, 28 bp, synthetic construct
  source 1..28: mol_type = other DNA
atatcctttaacacaaccagctctgcgg

SEQ ID NO: 26081 - DNA, 28 bp, synthetic construct
  source 1..28: mol_type = other DNA
tgcaatatgaatgcatgactccacaagg

SEQ ID NO: 26082 - DNA, 28 bp, synthetic construct
  source 1..28: mol_type = other DNA
tgcatgactccacaaggctttcctgtgg

SEQ ID NO: 26083 - DNA, 28 bp, synthetic construct
  source 1..28: mol_type = other DNA
gcatgactccacaaggctttcctgtggg

SEQ ID NO: 26084 - DNA, 28 bp, synthetic construct
  source 1..28: mol_type = other DNA
tgggcaggcccacaggaaagccttgtgg

SEQ ID NO: 26085 - DNA, 28 bp, synthetic construct
  source 1..28: mol_type = other DNA
aggctttcctgtgggcctgcccagatgg

SEQ ID NO: 26086 - DNA, 28 bp, synthetic construct
  source 1..28: mol_type = other DNA
tcctgtgggcctgcccagatggacctgg

SEQ ID NO: 26087 - DNA, 28 bp, synthetic construct
  source 1..28: mol_type = other DNA
accaggtccatctgggcaggcccacagg

SEQ ID NO: 26088 - DNA, 28 bp, synthetic construct
  source 1..28: mol_type = other DNA
tgtgggcctgcccagatggacctggtgg

SEQ ID NO: 26089 - DNA, 28 bp, synthetic construct
  source 1..28: mol_type = other DNA
gtgcatccaccaggtccatctgggcagg

SEQ ID NO: 26090 - DNA, 28 bp, synthetic construct
  source 1..28: mol_type = other DNA
ggaggtgcatccaccaggtccatctggg

SEQ ID NO: 26091 - DNA, 28 bp, synthetic construct
  source 1..28: mol_type = other DNA
tggaggtgcatccaccaggtccatctgg

SEQ ID NO: 26092 - DNA, 28 bp, synthetic construct
  source 1..28: mol_type = other DNA
gatggacctggtggatgcacctccatgg

SEQ ID NO: 26093 - DNA, 28 bp, synthetic construct
  source 1..28: mol_type = other DNA
tggcagccatggaggtgcatccaccagg

SEQ ID NO: 26094 - DNA, 28 bp, synthetic construct
  source 1..28: mol_type = other DNA
gatgcacctccatggctgccatgagtgg

SEQ ID NO: 26095 - DNA, 28 bp, synthetic construct
  source 1..28: mol_type = other DNA
cactgaccactcatggcagccatggagg

SEQ ID NO: 26096 - DNA, 28 bp, synthetic construct
  source 1..28: mol_type = other DNA
tgtcactgaccactcatggcagccatgg

SEQ ID NO: 26097 - DNA, 28 bp, synthetic construct
  source 1..28: mol_type = other DNA
cctatgtcttgtcactgaccactcatgg

SEQ ID NO: 26098 - DNA, 28 bp, synthetic construct
  source 1..28: mol_type = other DNA
gtggtcagtgacaagacataggctaagg

SEQ ID NO: 26099 - DNA, 28 bp, synthetic construct
  source 1..28: mol_type = other DNA
tcagtgacaagacataggctaaggctgg

SEQ ID NO: 26100 - DNA, 28 bp, synthetic construct
  source 1..28: mol_type = other DNA
gacaagacataggctaaggctggcatgg

SEQ ID NO: 26101 - DNA, 28 bp, synthetic construct
  source 1..28: mol_type = other DNA
acaagacataggctaaggctggcatggg

SEQ ID NO: 26102 - DNA, 28 bp, synthetic construct
  source 1..28: mol_type = other DNA
caagacataggctaaggctggcatgggg

SEQ ID NO: 26103 - DNA, 28 bp, synthetic construct
  source 1..28: mol_type = other DNA
cataggctaaggctggcatggggactgg

SEQ ID NO: 26104 - DNA, 28 bp, synthetic construct
  source 1..28: mol_type = other DNA
ggggactggagtgcatcccagtccccgg

SEQ ID NO: 26105 - DNA, 28 bp, synthetic construct
  source 1..28: mol_type = other DNA
cttcacaagaggatggccggggactggg

SEQ ID NO: 26106 - DNA, 28 bp, synthetic construct
  source 1..28: mol_type = other DNA
ccagtccccggccatcctcttgtgaagg

SEQ ID NO: 26107 - DNA, 28 bp, synthetic construct
  source 1..28: mol_type = other DNA
gacagccttcacaagaggatggccgggg

SEQ ID NO: 26108 - DNA, 28 bp, synthetic construct
  source 1..28: mol_type = other DNA
tgacagccttcacaagaggatggccggg

SEQ ID NO: 26109 - DNA, 28 bp, synthetic construct
  source 1..28: mol_type = other DNA
ttgacagccttcacaagaggatggccgg

SEQ ID NO: 26110 - DNA, 28 bp, synthetic construct
  source 1..28: mol_type = other DNA
ggccatcctcttgtgaaggctgtcaagg

SEQ ID NO: 26111 - DNA, 28 bp, synthetic construct
  source 1..28: mol_type = other DNA
caccttgacagccttcacaagaggatgg

SEQ ID NO: 26112 - DNA, 28 bp, synthetic construct
  source 1..28: mol_type = other DNA
catcctcttgtgaaggctgtcaaggtgg

SEQ ID NO: 26113 - DNA, 28 bp, synthetic construct
  source 1..28: mol_type = other DNA
atcctcttgtgaaggctgtcaaggtggg

SEQ ID NO: 26114 - DNA, 28 bp, synthetic construct
  source 1..28: mol_type = other DNA
tcctcttgtgaaggctgtcaaggtgggg

SEQ ID NO: 26115 - DNA, 28 bp, synthetic construct
  source 1..28: mol_type = other DNA
tccccaccttgacagccttcacaagagg

SEQ ID NO: 26116 - DNA, 28 bp, synthetic construct
  source 1..28: mol_type = other DNA
tttgagtcatatgcagatgaaacctagg

SEQ ID NO: 26117 - DNA, 28 bp, synthetic construct
  source 1..28: mol_type = other DNA
catatgcagatgaaacctaggctgctgg

SEQ ID NO: 26118 - DNA, 28 bp, synthetic construct
  source 1..28: mol_type = other DNA
atatgcagatgaaacctaggctgctggg

SEQ ID NO: 26119 - DNA, 28 bp, synthetic construct
  source 1..28: mol_type = other DNA
ggtaacaaagacaacccagcagcctagg

SEQ ID NO: 26120 - DNA, 28 bp, synthetic construct
  source 1..28: mol_type = other DNA
tctttgttaccttgcctctctgttgagg

SEQ ID NO: 26121 - DNA, 28 bp, synthetic construct
  source 1..28: mol_type = other DNA
ctatcacatcctcaacagagaggcaagg

SEQ ID NO: 26122 - DNA, 28 bp, synthetic construct
  source 1..28: mol_type = other DNA
tgctgctatcacatcctcaacagagagg

SEQ ID NO: 26123 - DNA, 28 bp, synthetic construct
  source 1..28: mol_type = other DNA
tgaggatgtgatagcagcacctaacagg

SEQ ID NO: 26124 - DNA, 28 bp, synthetic construct
  source 1..28: mol_type = other DNA
aggggaggcaggctatgaacctgttagg

SEQ ID NO: 26125 - DNA, 28 bp, synthetic construct
  source 1..28: mol_type = other DNA
acattgggagaagaggaggggaggcagg

SEQ ID NO: 26126 - DNA, 28 bp, synthetic construct
  source 1..28: mol_type = other DNA
aatgacattgggagaagaggaggggagg

SEQ ID NO: 26127 - DNA, 28 bp, synthetic construct
  source 1..28: mol_type = other DNA
tgaaatgacattgggagaagaggagggg

SEQ ID NO: 26128 - DNA, 28 bp, synthetic construct
  source 1..28: mol_type = other DNA
gtgaaatgacattgggagaagaggaggg

SEQ ID NO: 26129 - DNA, 28 bp, synthetic construct
  source 1..28: mol_type = other DNA
tgtgaaatgacattgggagaagaggagg

SEQ ID NO: 26130 - DNA, 28 bp, synthetic construct
  source 1..28: mol_type = other DNA
aactgtgaaatgacattgggagaagagg

SEQ ID NO: 26131 - DNA, 28 bp, synthetic construct
  source 1..28: mol_type = other DNA
aaacattaaactgtgaaatgacattggg

SEQ ID NO: 26132 - DNA, 28 bp, synthetic construct
  source 1..28: mol_type = other DNA
taaacattaaactgtgaaatgacattgg

SEQ ID NO: 26133 - DNA, 28 bp, synthetic construct
  source 1..28: mol_type = other DNA
ttaatgtttaagcgtatgtttaagatgg

SEQ ID NO: 26134 - DNA, 28 bp, synthetic construct
  source 1..28: mol_type = other DNA
atgggaacaataggttgcatcttattgg

SEQ ID NO: 26135 - DNA, 28 bp, synthetic construct
  source 1..28: mol_type = other DNA
atgcaacctattgttcccatgcttttgg

SEQ ID NO: 26136 - DNA, 28 bp, synthetic construct
  source 1..28: mol_type = other DNA
aatttaccaaaagcatgggaacaatagg

SEQ ID NO: 26137 - DNA, 28 bp, synthetic construct
  source 1..28: mol_type = other DNA
gacaaatttaatttaccaaaagcatggg

SEQ ID NO: 26138 - DNA, 28 bp, synthetic construct
  source 1..28: mol_type = other DNA
agacaaatttaatttaccaaaagcatgg

SEQ ID NO: 26139 - DNA, 28 bp, synthetic construct
  source 1..28: mol_type = other DNA
aatttgtctgattgcagtatttacaagg

SEQ ID NO: 26140 - DNA, 28 bp, synthetic construct
  source 1..28: mol_type = other DNA
caaataaagacactcaacatttaaaagg

SEQ ID NO: 26141 - DNA, 28 bp, synthetic construct
  source 1..28: mol_type = other DNA
caataaaagactaacactttagacaagg

SEQ ID NO: 26142 - DNA, 28 bp, synthetic construct
  source 1..28: mol_type = other DNA
tgccacgagccttgcaaagcctgacagg

SEQ ID NO: 26143 - DNA, 28 bp, synthetic construct
  source 1..28: mol_type = other DNA
atcctgtcaggctttgcaaggctcgtgg

SEQ ID NO: 26144 - DNA, 28 bp, synthetic construct
  source 1..28: mol_type = other DNA
ggaaaatatcctgtcaggctttgcaagg

SEQ ID NO: 26145 - DNA, 28 bp, synthetic construct
  source 1..28: mol_type = other DNA
agttgtcatgtattcagtccacttaagg

SEQ ID NO: 26146 - DNA, 28 bp, synthetic construct
  source 1..28: mol_type = other DNA
gttgtcatgtattcagtccacttaaggg

SEQ ID NO: 26147 - DNA, 28 bp, synthetic construct
  source 1..28: mol_type = other DNA
atgtattcagtccacttaagggcagtgg

SEQ ID NO: 26148 - DNA, 28 bp, synthetic construct
  source 1..28: mol_type = other DNA
tgtattcagtccacttaagggcagtggg

SEQ ID NO: 26149 - DNA, 28 bp, synthetic construct
  source 1..28: mol_type = other DNA
gtattcagtccacttaagggcagtgggg

SEQ ID NO: 26150 - DNA, 28 bp, synthetic construct
  source 1..28: mol_type = other DNA
caaacgcttccccactgcccttaagtgg

SEQ ID NO: 26151 - DNA, 28 bp, synthetic construct
  source 1..28: mol_type = other DNA
aagggcagtggggaagcgtttgagacgg

SEQ ID NO: 26152 - DNA, 28 bp, synthetic construct
  source 1..28: mol_type = other DNA
tggggaagcgtttgagacggagctgtgg

SEQ ID NO: 26153 - DNA, 28 bp, synthetic construct
  source 1..28: mol_type = other DNA
ggaagcgtttgagacggagctgtggagg

SEQ ID NO: 26154 - DNA, 28 bp, synthetic construct
  source 1..28: mol_type = other DNA
ggagctgtggaggctgaatccttgaagg

SEQ ID NO: 26155 - DNA, 28 bp, synthetic construct
  source 1..28: mol_type = other DNA
gctgtggaggctgaatccttgaaggagg

SEQ ID NO: 26156 - DNA, 28 bp, synthetic construct
  source 1..28: mol_type = other DNA
gtggaggctgaatccttgaaggaggagg

SEQ ID NO: 26157 - DNA, 28 bp, synthetic construct
  source 1..28: mol_type = other DNA
gaatccttgaaggaggaggtgagagagg

SEQ ID NO: 26158 - DNA, 28 bp, synthetic construct
  source 1..28: mol_type = other DNA
tgtgcctctctcacctcctccttcaagg

SEQ ID NO: 26159 - DNA, 28 bp, synthetic construct
  source 1..28: mol_type = other DNA
ttgaaggaggaggtgagagaggcacagg

SEQ ID NO: 26160 - DNA, 28 bp, synthetic construct
  source 1..28: mol_type = other DNA
cgggagagaagaggggacatgcactggg

SEQ ID NO: 26161 - DNA, 28 bp, synthetic construct
  source 1..28: mol_type = other DNA
tcgggagagaagaggggacatgcactgg

SEQ ID NO: 26162 - DNA, 28 bp, synthetic construct
  source 1..28: mol_type = other DNA
atgacactgcatcgggagagaagagggg

SEQ ID NO: 26163 - DNA, 28 bp, synthetic construct
  source 1..28: mol_type = other DNA
aatgacactgcatcgggagagaagaggg

SEQ ID NO: 26164 - DNA, 28 bp, synthetic construct
  source 1..28: mol_type = other DNA
gaatgacactgcatcgggagagaagagg

SEQ ID NO: 26165 - DNA, 28 bp, synthetic construct
  source 1..28: mol_type = other DNA
tctctcccgatgcagtgtcattcccagg

SEQ ID NO: 26166 - DNA, 28 bp, synthetic construct
  source 1..28: mol_type = other DNA
gttcacctgggaatgacactgcatcggg

SEQ ID NO: 26167 - DNA, 28 bp, synthetic construct
  source 1..28: mol_type = other DNA
ggttcacctgggaatgacactgcatcgg

SEQ ID NO: 26168 - DNA, 28 bp, synthetic construct
  source 1..28: mol_type = other DNA
cagtgtcattcccaggtgaacctgccgg

SEQ ID NO: 26169 - DNA, 28 bp, synthetic construct
  source 1..28: mol_type = other DNA
agtgtcattcccaggtgaacctgccggg

SEQ ID NO: 26170 - DNA, 28 bp, synthetic construct
  source 1..28: mol_type = other DNA
tcccaggtgaacctgccgggctgaacgg

SEQ ID NO: 26171 - DNA, 28 bp, synthetic construct
  source 1..28: mol_type = other DNA
gccgttcagcccggcaggttcacctggg

SEQ ID NO: 26172 - DNA, 28 bp, synthetic construct
  source 1..28: mol_type = other DNA
ggccgttcagcccggcaggttcacctgg

SEQ ID NO: 26173 - DNA, 28 bp, synthetic construct
  source 1..28: mol_type = other DNA
ggtgaacctgccgggctgaacggcctgg

SEQ ID NO: 26174 - DNA, 28 bp, synthetic construct
  source 1..28: mol_type = other DNA
gaggggccaggccgttcagcccggcagg

SEQ ID NO: 26175 - DNA, 28 bp, synthetic construct
  source 1..28: mol_type = other DNA
aatagaggggccaggccgttcagcccgg

SEQ ID NO: 26176 - DNA, 28 bp, synthetic construct
  source 1..28: mol_type = other DNA
gaacggcctggcccctctattcagtcgg

SEQ ID NO: 26177 - DNA, 28 bp, synthetic construct
  source 1..28: mol_type = other DNA
aaaactccgactgaatagaggggccagg

SEQ ID NO: 26178 - DNA, 28 bp, synthetic construct
  source 1..28: mol_type = other DNA
gtagtaaaactccgactgaatagagggg

SEQ ID NO: 26179 - DNA, 28 bp, synthetic construct
  source 1..28: mol_type = other DNA
agtagtaaaactccgactgaatagaggg

SEQ ID NO: 26180 - DNA, 28 bp, synthetic construct
  source 1..28: mol_type = other DNA
gagtagtaaaactccgactgaatagagg

SEQ ID NO: 26181 - DNA, 28 bp, synthetic construct
  source 1..28: mol_type = other DNA
ttcagtcggagttttactactccagtgg

SEQ ID NO: 26182 - DNA, 28 bp, synthetic construct
  source 1..28: mol_type = other DNA
aaaactattaaaataaatacaatcaggg

SEQ ID NO: 26183 - DNA, 28 bp, synthetic construct
  source 1..28: mol_type = other DNA
aaaaactattaaaataaatacaatcagg

SEQ ID NO: 26184 - DNA, 28 bp, synthetic construct
  source 1..28: mol_type = other DNA
agttttttaaaaaacgcttgtaatcagg

SEQ ID NO: 26185 - DNA, 28 bp, synthetic construct
  source 1..28: mol_type = other DNA
tctgtcttttttatattacccagtttgg

SEQ ID NO: 26186 - DNA, 28 bp, synthetic construct
  source 1..28: mol_type = other DNA
ctgtcttttttatattacccagtttggg

SEQ ID NO: 26187 - DNA, 28 bp, synthetic construct
  source 1..28: mol_type = other DNA
ttttttatattacccagtttgggagtgg

SEQ ID NO: 26188 - DNA, 28 bp, synthetic construct
  source 1..28: mol_type = other DNA
atttaagttctgccactcccaaactggg

SEQ ID NO: 26189 - DNA, 28 bp, synthetic construct
  source 1..28: mol_type = other DNA
catttaagttctgccactcccaaactgg

SEQ ID NO: 26190 - DNA, 28 bp, synthetic construct
  source 1..28: mol_type = other DNA
acagtggttcttaatcaggtggaagagg

SEQ ID NO: 26191 - DNA, 28 bp, synthetic construct
  source 1..28: mol_type = other DNA
tctgctacagtggttcttaatcaggtgg

SEQ ID NO: 26192 - DNA, 28 bp, synthetic construct
  source 1..28: mol_type = other DNA
gcgtctgctacagtggttcttaatcagg

SEQ ID NO: 26193 - DNA, 28 bp, synthetic construct
  source 1..28: mol_type = other DNA
accactgtagcagacgcagacttattgg

SEQ ID NO: 26194 - DNA, 28 bp, synthetic construct
  source 1..28: mol_type = other DNA
tccaataagtctgcgtctgctacagtgg

SEQ ID NO: 26195 - DNA, 28 bp, synthetic construct
  source 1..28: mol_type = other DNA
agcagacgcagacttattggacactagg

SEQ ID NO: 26196 - DNA, 28 bp, synthetic construct
  source 1..28: mol_type = other DNA
agacgcagacttattggacactaggcgg

SEQ ID NO: 26197 - DNA, 28 bp, synthetic construct
  source 1..28: mol_type = other DNA
gacgcagacttattggacactaggcggg

SEQ ID NO: 26198 - DNA, 28 bp, synthetic construct
  source 1..28: mol_type = other DNA
gcagacttattggacactaggcgggagg

SEQ ID NO: 26199 - DNA, 28 bp, synthetic construct
  source 1..28: mol_type = other DNA
gcgggaggccagctctgcagacagcagg

SEQ ID NO: 26200 - DNA, 28 bp, synthetic construct
  source 1..28: mol_type = other DNA
gccagctctgcagacagcaggtctcagg

SEQ ID NO: 26201 - DNA, 28 bp, synthetic construct
  source 1..28: mol_type = other DNA
tcctgagacctgctgtctgcagagctgg

SEQ ID NO: 26202 - DNA, 28 bp, synthetic construct
  source 1..28: mol_type = other DNA
ctgcagacagcaggtctcaggaagacgg

SEQ ID NO: 26203 - DNA, 28 bp, synthetic construct
  source 1..28: mol_type = other DNA
acagcaggtctcaggaagacggtcaagg

SEQ ID NO: 26204 - DNA, 28 bp, synthetic construct
  source 1..28: mol_type = other DNA
aggtctcaggaagacggtcaaggcatgg

SEQ ID NO: 26205 - DNA, 28 bp, synthetic construct
  source 1..28: mol_type = other DNA
ggcatggctgctgatgatccgcttatgg

SEQ ID NO: 26206 - DNA, 28 bp, synthetic construct
  source 1..28: mol_type = other DNA
gcatggctgctgatgatccgcttatggg

SEQ ID NO: 26207 - DNA, 28 bp, synthetic construct
  source 1..28: mol_type = other DNA
ctaagacaataaacacacccataagcgg

SEQ ID NO: 26208 - DNA, 28 bp, synthetic construct
  source 1..28: mol_type = other DNA
attgtcttagcccatgttagatgcgagg

SEQ ID NO: 26209 - DNA, 28 bp, synthetic construct
  source 1..28: mol_type = other DNA
gtgagtggttcctcgcatctaacatggg

SEQ ID NO: 26210 - DNA, 28 bp, synthetic construct
  source 1..28: mol_type = other DNA
tgtgagtggttcctcgcatctaacatgg

SEQ ID NO: 26211 - DNA, 28 bp, synthetic construct
  source 1..28: mol_type = other DNA
caggagctgtcatttgcagtgtgagtgg

SEQ ID NO: 26212 - DNA, 28 bp, synthetic construct
  source 1..28: mol_type = other DNA
cactcacactgcaaatgacagctcctgg

SEQ ID NO: 26213 - DNA, 28 bp, synthetic construct
  source 1..28: mol_type = other DNA
gcaagtatgacactaagactgagccagg

SEQ ID NO: 26214 - DNA, 28 bp, synthetic construct
  source 1..28: mol_type = other DNA
tcttagtgtcatacttgcctttaactgg

SEQ ID NO: 26215 - DNA, 28 bp, synthetic construct
  source 1..28: mol_type = other DNA
gtattgcaggggagttgccagttaaagg

SEQ ID NO: 26216 - DNA, 28 bp, synthetic construct
  source 1..28: mol_type = other DNA
ttaactggcaactcccctgcaatacagg

SEQ ID NO: 26217 - DNA, 28 bp, synthetic construct
  source 1..28: mol_type = other DNA
taactggcaactcccctgcaatacaggg

SEQ ID NO: 26218 - DNA, 28 bp, synthetic construct
  source 1..28: mol_type = other DNA
gaggtgcctttcatggtgattaagatgg

SEQ ID NO: 26219 - DNA, 28 bp, synthetic construct
  source 1..28: mol_type = other DNA
aggtgcctttcatggtgattaagatggg

SEQ ID NO: 26220 - DNA, 28 bp, synthetic construct
  source 1..28: mol_type = other DNA
ccaatcccatcttaatcaccatgaaagg

SEQ ID NO: 26221 - DNA, 28 bp, synthetic construct
  source 1..28: mol_type = other DNA
atgggattggttgttcacttaaatatgg

SEQ ID NO: 26222 - DNA, 28 bp, synthetic construct
  source 1..28: mol_type = other DNA
tgggattggttgttcacttaaatatggg

SEQ ID NO: 26223 - DNA, 28 bp, synthetic construct
  source 1..28: mol_type = other DNA
tcccacccctccccacccccaaattagg

SEQ ID NO: 26224 - DNA, 28 bp, synthetic construct
  source 1..28: mol_type = other DNA
ccctaatttgggggtggggaggggtggg

SEQ ID NO: 26225 - DNA, 28 bp, synthetic construct
  source 1..28: mol_type = other DNA
tccctaatttgggggtggggaggggtgg

SEQ ID NO: 26226 - DNA, 28 bp, synthetic construct
  source 1..28: mol_type = other DNA
ttctccctaatttgggggtggggagggg

SEQ ID NO: 26227 - DNA, 28 bp, synthetic construct
  source 1..28: mol_type = other DNA
tttctccctaatttgggggtggggaggg

SEQ ID NO: 26228 - DNA, 28 bp, synthetic construct
  source 1..28: mol_type = other DNA
gtttctccctaatttgggggtggggagg

SEQ ID NO: 26229 - DNA, 28 bp, synthetic construct
  source 1..28: mol_type = other DNA
ttagtttctccctaatttgggggtgggg

SEQ ID NO: 26230 - DNA, 28 bp, synthetic construct
  source 1..28: mol_type = other DNA
cttagtttctccctaatttgggggtggg

SEQ ID NO: 26231 - DNA, 28 bp, synthetic construct
  source 1..28: mol_type = other DNA
tcttagtttctccctaatttgggggtgg

SEQ ID NO: 26232 - DNA, 28 bp, synthetic construct
  source 1..28: mol_type = other DNA
gcttcttagtttctccctaatttggggg

SEQ ID NO: 26233 - DNA, 28 bp, synthetic construct
  source 1..28: mol_type = other DNA
agcttcttagtttctccctaatttgggg

SEQ ID NO: 26234 - DNA, 28 bp, synthetic construct
  source 1..28: mol_type = other DNA
aagcttcttagtttctccctaatttggg

SEQ ID NO: 26235 - DNA, 28 bp, synthetic construct
  source 1..28: mol_type = other DNA
aaagcttcttagtttctccctaatttgg

SEQ ID NO: 26236 - DNA, 28 bp, synthetic construct
  source 1..28: mol_type = other DNA
taagaagctttccttttgttgtttcagg

SEQ ID NO: 26237 - DNA, 28 bp, synthetic construct
  source 1..28: mol_type = other DNA
attcaaaaatacctgaaacaacaaaagg

SEQ ID NO: 26238 - DNA, 28 bp, synthetic construct
  source 1..28: mol_type = other DNA
cgactgttacgttacattgtccgcctgg

SEQ ID NO: 26239 - DNA, 28 bp, synthetic construct
  source 1..28: mol_type = other DNA
gttacgttacattgtccgcctggtgtgg

SEQ ID NO: 26240 - DNA, 28 bp, synthetic construct
  source 1..28: mol_type = other DNA
ctgtcaatgcattctccacaccaggcgg

SEQ ID NO: 26241 - DNA, 28 bp, synthetic construct
  source 1..28: mol_type = other DNA
cgcctggtgtggagaatgcattgacagg

SEQ ID NO: 26242 - DNA, 28 bp, synthetic construct
  source 1..28: mol_type = other DNA
aacctgtcaatgcattctccacaccagg

SEQ ID NO: 26243 - DNA, 28 bp, synthetic construct
  source 1..28: mol_type = other DNA
ggagaatgcattgacaggttctttgcgg

SEQ ID NO: 26244 - DNA, 28 bp, synthetic construct
  source 1..28: mol_type = other DNA
caagcaaaatgtctgcatggtatctcgg

SEQ ID NO: 26245 - DNA, 28 bp, synthetic construct
  source 1..28: mol_type = other DNA
ggtttgaacaagcaaaatgtctgcatgg

SEQ ID NO: 26246 - DNA, 28 bp, synthetic construct
  source 1..28: mol_type = other DNA
ttcaaaccaacaagacccagcaccgcgg

SEQ ID NO: 26247 - DNA, 28 bp, synthetic construct
  source 1..28: mol_type = other DNA
aggagaccgcggtgctgggtcttgttgg

SEQ ID NO: 26248 - DNA, 28 bp, synthetic construct
  source 1..28: mol_type = other DNA
aacaagacccagcaccgcggtctcctgg

SEQ ID NO: 26249 - DNA, 28 bp, synthetic construct
  source 1..28: mol_type = other DNA
aatggcaccaggagaccgcggtgctggg

SEQ ID NO: 26250 - DNA, 28 bp, synthetic construct
  source 1..28: mol_type = other DNA
taatggcaccaggagaccgcggtgctgg

SEQ ID NO: 26251 - DNA, 28 bp, synthetic construct
  source 1..28: mol_type = other DNA
gcataataatggcaccaggagaccgcgg

SEQ ID NO: 26252 - DNA, 28 bp, synthetic construct
  source 1..28: mol_type = other DNA
ccgctggctgcataataatggcaccagg

SEQ ID NO: 26253 - DNA, 28 bp, synthetic construct
  source 1..28: mol_type = other DNA
aagagaaccgctggctgcataataatgg

SEQ ID NO: 26254 - DNA, 28 bp, synthetic construct
  source 1..28: mol_type = other DNA
tattatgcagccagcggttctcttgtgg

SEQ ID NO: 26255 - DNA, 28 bp, synthetic construct
  source 1..28: mol_type = other DNA
tatgcagccagcggttctcttgtggagg

SEQ ID NO: 26256 - DNA, 28 bp, synthetic construct
  source 1..28: mol_type = other DNA
atgcagccagcggttctcttgtggaggg

SEQ ID NO: 26257 - DNA, 28 bp, synthetic construct
  source 1..28: mol_type = other DNA
tgcagccagcggttctcttgtggagggg

SEQ ID NO: 26258 - DNA, 28 bp, synthetic construct
  source 1..28: mol_type = other DNA
gcagccagcggttctcttgtggaggggg

SEQ ID NO: 26259 - DNA, 28 bp, synthetic construct
  source 1..28: mol_type = other DNA
ccagcggttctcttgtggagggggcagg

SEQ ID NO: 26260 - DNA, 28 bp, synthetic construct
  source 1..28: mol_type = other DNA
ggtgacgtttcagaagacaccgagctgg

SEQ ID NO: 26261 - DNA, 28 bp, synthetic construct
  source 1..28: mol_type = other DNA
acgtttcagaagacaccgagctggatgg

SEQ ID NO: 26262 - DNA, 28 bp, synthetic construct
  source 1..28: mol_type = other DNA
cgtttcagaagacaccgagctggatggg

SEQ ID NO: 26263 - DNA, 28 bp, synthetic construct
  source 1..28: mol_type = other DNA
aacagaaaggtagtcccatccagctcgg

SEQ ID NO: 26264 - DNA, 28 bp, synthetic construct
  source 1..28: mol_type = other DNA
ttctgctgtgtggtgatgaacagaaagg

SEQ ID NO: 26265 - DNA, 28 bp, synthetic construct
  source 1..28: mol_type = other DNA
catcaccacacagcagaatttctaatgg

SEQ ID NO: 26266 - DNA, 28 bp, synthetic construct
  source 1..28: mol_type = other DNA
aacttccattagaaattctgctgtgtgg

SEQ ID NO: 26267 - DNA, 28 bp, synthetic construct
  source 1..28: mol_type = other DNA
taatggaagtttgttgtgaatgtaaagg

SEQ ID NO: 26268 - DNA, 28 bp, synthetic construct
  source 1..28: mol_type = other DNA
tggaagtttgttgtgaatgtaaaggagg

SEQ ID NO: 26269 - DNA, 28 bp, synthetic construct
  source 1..28: mol_type = other DNA
ggaagtttgttgtgaatgtaaaggaggg

SEQ ID NO: 26270 - DNA, 28 bp, synthetic construct
  source 1..28: mol_type = other DNA
tctttgctttttaatatacaaaccatgg

SEQ ID NO: 26271 - DNA, 28 bp, synthetic construct
  source 1..28: mol_type = other DNA
ttttaatatacaaaccatggttttttgg

SEQ ID NO: 26272 - DNA, 28 bp, synthetic construct
  source 1..28: mol_type = other DNA
tatacaaaccatggttttttggagcagg

SEQ ID NO: 26273 - DNA, 28 bp, synthetic construct
  source 1..28: mol_type = other DNA
cacaaaatcctgctccaaaaaaccatgg

SEQ ID NO: 26274 - DNA, 28 bp, synthetic construct
  source 1..28: mol_type = other DNA
tttggagcaggattttgtgtaagaatgg

SEQ ID NO: 26275 - DNA, 28 bp, synthetic construct
  source 1..28: mol_type = other DNA
tgtgttttccccctcaccttcaataagg

SEQ ID NO: 26276 - DNA, 28 bp, synthetic construct
  source 1..28: mol_type = other DNA
ttgaaaaaccttattgaaggtgaggggg

SEQ ID NO: 26277 - DNA, 28 bp, synthetic construct
  source 1..28: mol_type = other DNA
tttgaaaaaccttattgaaggtgagggg

SEQ ID NO: 26278 - DNA, 28 bp, synthetic construct
  source 1..28: mol_type = other DNA
ttttgaaaaaccttattgaaggtgaggg

SEQ ID NO: 26279 - DNA, 28 bp, synthetic construct
  source 1..28: mol_type = other DNA
tttttgaaaaaccttattgaaggtgagg

SEQ ID NO: 26280 - DNA, 28 bp, synthetic construct
  source 1..28: mol_type = other DNA
tcaccttcaataaggtttttcaaaaagg

SEQ ID NO: 26281 - DNA, 28 bp, synthetic construct
  source 1..28: mol_type = other DNA
tttcctttttgaaaaaccttattgaagg

SEQ ID NO: 26282 - DNA, 28 bp, synthetic construct
  source 1..28: mol_type = other DNA
tcaataaggtttttcaaaaaggaaatgg

SEQ ID NO: 26283 - DNA, 28 bp, synthetic construct
  source 1..28: mol_type = other DNA
tttaatacaaaagttattcacaaattgg

SEQ ID NO: 26284 - DNA, 28 bp, synthetic construct
  source 1..28: mol_type = other DNA
tttgtattaaaattttaagaacctacgg

SEQ ID NO: 26285 - DNA, 28 bp, synthetic construct
  source 1..28: mol_type = other DNA
ttaagaacctacggcctattctcagagg

SEQ ID NO: 26286 - DNA, 28 bp, synthetic construct
  source 1..28: mol_type = other DNA
acataatcctctgagaataggccgtagg

SEQ ID NO: 26287 - DNA, 28 bp, synthetic construct
  source 1..28: mol_type = other DNA
aggggttacataatcctctgagaatagg

SEQ ID NO: 26288 - DNA, 28 bp, synthetic construct
  source 1..28: mol_type = other DNA
tcagaggattatgtaacccctgcagtgg

SEQ ID NO: 26289 - DNA, 28 bp, synthetic construct
  source 1..28: mol_type = other DNA
ttagctggctcagtttccactgcagggg

SEQ ID NO: 26290 - DNA, 28 bp, synthetic construct
  source 1..28: mol_type = other DNA
gttagctggctcagtttccactgcaggg

SEQ ID NO: 26291 - DNA, 28 bp, synthetic construct
  source 1..28: mol_type = other DNA
agttagctggctcagtttccactgcagg

SEQ ID NO: 26292 - DNA, 28 bp, synthetic construct
  source 1..28: mol_type = other DNA
aactaaggcagctttttaagttagctgg

SEQ ID NO: 26293 - DNA, 28 bp, synthetic construct
  source 1..28: mol_type = other DNA
ttctgtaatctctaaaaataaactaagg

SEQ ID NO: 26294 - DNA, 28 bp, synthetic construct
  source 1..28: mol_type = other DNA
tttagagattacagaatttttaaacagg

SEQ ID NO: 26295 - DNA, 28 bp, synthetic construct
  source 1..28: mol_type = other DNA
ttagagattacagaatttttaaacaggg

SEQ ID NO: 26296 - DNA, 28 bp, synthetic construct
  source 1..28: mol_type = other DNA
cagagaggcaatagtagggaagggaggg

SEQ ID NO: 26297 - DNA, 28 bp, synthetic construct
  source 1..28: mol_type = other DNA
tcagagaggcaatagtagggaagggagg

SEQ ID NO: 26298 - DNA, 28 bp, synthetic construct
  source 1..28: mol_type = other DNA
aggtcagagaggcaatagtagggaaggg

SEQ ID NO: 26299 - DNA, 28 bp, synthetic construct
  source 1..28: mol_type = other DNA
aaggtcagagaggcaatagtagggaagg

SEQ ID NO: 26300 - DNA, 28 bp, synthetic construct
  source 1..28: mol_type = other DNA
taaaaaggtcagagaggcaatagtaggg

SEQ ID NO: 26301 - DNA, 28 bp, synthetic construct
  source 1..28: mol_type = other DNA
ttaaaaaggtcagagaggcaatagtagg

SEQ ID NO: 26302 - DNA, 28 bp, synthetic construct
  source 1..28: mol_type = other DNA
taaaaataatttaaaaaggtcagagagg

SEQ ID NO: 26303 - DNA, 28 bp, synthetic construct
  source 1..28: mol_type = other DNA
ttttggtattaaaaataatttaaaaagg

SEQ ID NO: 26304 - DNA, 28 bp, synthetic construct
  source 1..28: mol_type = other DNA
taataccaaaagagttcttttgaaatgg

SEQ ID NO: 26305 - DNA, 28 bp, synthetic construct
  source 1..28: mol_type = other DNA
cagttccatttcaaaagaactcttttgg

SEQ ID NO: 26306 - DNA, 28 bp, synthetic construct
  source 1..28: mol_type = other DNA
ttcttttgaaatggaactgattaaaagg

SEQ ID NO: 26307 - DNA, 28 bp, synthetic construct
  source 1..28: mol_type = other DNA
tcttttgaaatggaactgattaaaaggg

SEQ ID NO: 26308 - DNA, 28 bp, synthetic construct
  source 1..28: mol_type = other DNA
gaaatggaactgattaaaagggcagagg

SEQ ID NO: 26309 - DNA, 28 bp, synthetic construct
  source 1..28: mol_type = other DNA
aaatggaactgattaaaagggcagaggg

SEQ ID NO: 26310 - DNA, 28 bp, synthetic construct
  source 1..28: mol_type = other DNA
atgggactggtatatcaatgcaggctgg

SEQ ID NO: 26311 - DNA, 28 bp, synthetic construct
  source 1..28: mol_type = other DNA
acaaatgggactggtatatcaatgcagg

SEQ ID NO: 26312 - DNA, 28 bp, synthetic construct
  source 1..28: mol_type = other DNA
gtacgtaaatatttacaaatgggactgg

SEQ ID NO: 26313 - DNA, 28 bp, synthetic construct
  source 1..28: mol_type = other DNA
taaaggtacgtaaatatttacaaatggg

SEQ ID NO: 26314 - DNA, 28 bp, synthetic construct
  source 1..28: mol_type = other DNA
ataaaggtacgtaaatatttacaaatgg

SEQ ID NO: 26315 - DNA, 28 bp, synthetic construct
  source 1..28: mol_type = other DNA
acctttataaattcagttgcatctgtgg

SEQ ID NO: 26316 - DNA, 28 bp, synthetic construct
  source 1..28: mol_type = other DNA
gccacagatgcaactgaatttataaagg

SEQ ID NO: 26317 - DNA, 28 bp, synthetic construct
  source 1..28: mol_type = other DNA
tggagttgcatcacaaaaagtgatgagg

SEQ ID NO: 26318 - DNA, 28 bp, synthetic construct
  source 1..28: mol_type = other DNA
cactttttgtgatgcaactccagtctgg

SEQ ID NO: 26319 - DNA, 28 bp, synthetic construct
  source 1..28: mol_type = other DNA
caaatctatgcatctgagtccagactgg

SEQ ID NO: 26320 - DNA, 28 bp, synthetic construct
  source 1..28: mol_type = other DNA
cagtctggactcagatgcatagatttgg

SEQ ID NO: 26321 - DNA, 28 bp, synthetic construct
  source 1..28: mol_type = other DNA
atttcactttatcatgaaaatacactgg

SEQ ID NO: 26322 - DNA, 28 bp, synthetic construct
  source 1..28: mol_type = other DNA
agatcgctcgaactgtgcaagatacagg

SEQ ID NO: 26323 - DNA, 28 bp, synthetic construct
  source 1..28: mol_type = other DNA
acagttcgagcgatctgttattaactgg

SEQ ID NO: 26324 - DNA, 28 bp, synthetic construct
  source 1..28: mol_type = other DNA
cagttcgagcgatctgttattaactggg

SEQ ID NO: 26325 - DNA, 28 bp, synthetic construct
  source 1..28: mol_type = other DNA
gatctgttattaactgggaagcatttgg

SEQ ID NO: 26326 - DNA, 28 bp, synthetic construct
  source 1..28: mol_type = other DNA
ttattaactgggaagcatttggtgttgg

SEQ ID NO: 26327 - DNA, 28 bp, synthetic construct
  source 1..28: mol_type = other DNA
cattccatttcgacgagcatgttattgg

SEQ ID NO: 26328 - DNA, 28 bp, synthetic construct
  source 1..28: mol_type = other DNA
attccatttcgacgagcatgttattggg

SEQ ID NO: 26329 - DNA, 28 bp, synthetic construct
  source 1..28: mol_type = other DNA
cttcccaataacatgctcgtcgaaatgg

SEQ ID NO: 26330 - DNA, 28 bp, synthetic construct
  source 1..28: mol_type = other DNA
catgttattgggaagtattctgaagagg

SEQ ID NO: 26331 - DNA, 28 bp, synthetic construct
  source 1..28: mol_type = other DNA
taagtgctacgcccctttgtgctgctgg

SEQ ID NO: 26332 - DNA, 28 bp, synthetic construct
  source 1..28: mol_type = other DNA
cgcccctttgtgctgctggcttttctgg

SEQ ID NO: 26333 - DNA, 28 bp, synthetic construct
  source 1..28: mol_type = other DNA
aaccagaaaagccagcagcacaaagggg

SEQ ID NO: 26334 - DNA, 28 bp, synthetic construct
  source 1..28: mol_type = other DNA
caaccagaaaagccagcagcacaaaggg

SEQ ID NO: 26335 - DNA, 28 bp, synthetic construct
  source 1..28: mol_type = other DNA
gcaaccagaaaagccagcagcacaaagg

SEQ ID NO: 26336 - DNA, 28 bp, synthetic construct
  source 1..28: mol_type = other DNA
ttgtgctgctggcttttctggttgcagg

SEQ ID NO: 26337 - DNA, 28 bp, synthetic construct
  source 1..28: mol_type = other DNA
gcttttctggttgcaggctttcccatgg

SEQ ID NO: 26338 - DNA, 28 bp, synthetic construct
  source 1..28: mol_type = other DNA
tggttgcaggctttcccatggtcacagg

SEQ ID NO: 26339 - DNA, 28 bp, synthetic construct
  source 1..28: mol_type = other DNA
tgctgacagtgcatcctgtgaccatggg

SEQ ID NO: 26340 - DNA, 28 bp, synthetic construct
  source 1..28: mol_type = other DNA
atgctgacagtgcatcctgtgaccatgg

SEQ ID NO: 26341 - DNA, 28 bp, synthetic construct
  source 1..28: mol_type = other DNA
ggtcacaggatgcactgtcagcatcagg

SEQ ID NO: 26342 - DNA, 28 bp, synthetic construct
  source 1..28: mol_type = other DNA
atgcactgtcagcatcaggtcccagagg

SEQ ID NO: 26343 - DNA, 28 bp, synthetic construct
  source 1..28: mol_type = other DNA
tgcactgtcagcatcaggtcccagaggg

SEQ ID NO: 26344 - DNA, 28 bp, synthetic construct
  source 1..28: mol_type = other DNA
gctgtaatggacacggtggccctctggg

SEQ ID NO: 26345 - DNA, 28 bp, synthetic construct
  source 1..28: mol_type = other DNA
tgctgtaatggacacggtggccctctgg

SEQ ID NO: 26346 - DNA, 28 bp, synthetic construct
  source 1..28: mol_type = other DNA
ctggactctgctgtaatggacacggtgg

SEQ ID NO: 26347 - DNA, 28 bp, synthetic construct
  source 1..28: mol_type = other DNA
cagctggactctgctgtaatggacacgg

SEQ ID NO: 26348 - DNA, 28 bp, synthetic construct
  source 1..28: mol_type = other DNA
atgctgcagctggactctgctgtaatgg

SEQ ID NO: 26349 - DNA, 28 bp, synthetic construct
  source 1..28: mol_type = other DNA
gagggcgtgagctggatgctgcagctgg

SEQ ID NO: 26350 - DNA, 28 bp, synthetic construct
  source 1..28: mol_type = other DNA
ctgcagcatccagctcacgccctcatgg

SEQ ID NO: 26351 - DNA, 28 bp, synthetic construct
  source 1..28: mol_type = other DNA
tgcagcatccagctcacgccctcatggg

SEQ ID NO: 26352 - DNA, 28 bp, synthetic construct
  source 1..28: mol_type = other DNA
atccagctcacgccctcatgggaattgg

SEQ ID NO: 26353 - DNA, 28 bp, synthetic construct
  source 1..28: mol_type = other DNA
tgccaattcccatgagggcgtgagctgg

SEQ ID NO: 26354 - DNA, 28 bp, synthetic construct
  source 1..28: mol_type = other DNA
ctcacgccctcatgggaattggcacagg

SEQ ID NO: 26355 - DNA, 28 bp, synthetic construct
  source 1..28: mol_type = other DNA
gccctcatgggaattggcacaggcctgg

SEQ ID NO: 26356 - DNA, 28 bp, synthetic construct
  source 1..28: mol_type = other DNA
ccctcatgggaattggcacaggcctggg

SEQ ID NO: 26357 - DNA, 28 bp, synthetic construct
  source 1..28: mol_type = other DNA
cctcatgggaattggcacaggcctgggg

SEQ ID NO: 26358 - DNA, 28 bp, synthetic construct
  source 1..28: mol_type = other DNA
atgggaattggcacaggcctggggcagg

SEQ ID NO: 26359 - DNA, 28 bp, synthetic construct
  source 1..28: mol_type = other DNA
tgggaattggcacaggcctggggcaggg

SEQ ID NO: 26360 - DNA, 28 bp, synthetic construct
  source 1..28: mol_type = other DNA
cacaggcctggggcagggcttctgatgg

SEQ ID NO: 26361 - DNA, 28 bp, synthetic construct
  source 1..28: mol_type = other DNA
aaatggccatcagaagccctgccccagg

SEQ ID NO: 26362 - DNA, 28 bp, synthetic construct
  source 1..28: mol_type = other DNA
gcagggcttctgatggccatttgcttgg

SEQ ID NO: 26363 - DNA, 28 bp, synthetic construct
  source 1..28: mol_type = other DNA
actaaaatgcaggaggccaagcaaatgg

SEQ ID NO: 26364 - DNA, 28 bp, synthetic construct
  source 1..28: mol_type = other DNA
actgtgagttggactaaaatgcaggagg

SEQ ID NO: 26365 - DNA, 28 bp, synthetic construct
  source 1..28: mol_type = other DNA
tggactgtgagttggactaaaatgcagg

SEQ ID NO: 26366 - DNA, 28 bp, synthetic construct
  source 1..28: mol_type = other DNA
ggagtgaagctagtggactgtgagttgg

SEQ ID NO: 26367 - DNA, 28 bp, synthetic construct
  source 1..28: mol_type = other DNA
agtgaatttaaaggagtgaagctagtgg

SEQ ID NO: 26368 - DNA, 28 bp, synthetic construct
  source 1..28: mol_type = other DNA
cactcctttaaattcactttgaaacagg

SEQ ID NO: 26369 - DNA, 28 bp, synthetic construct
  source 1..28: mol_type = other DNA
gaggcctgtttcaaagtgaatttaaagg

SEQ ID NO: 26370 - DNA, 28 bp, synthetic construct
  source 1..28: mol_type = other DNA
ctatggtgctggtggaagtgggatgagg

SEQ ID NO: 26371 - DNA, 28 bp, synthetic construct
  source 1..28: mol_type = other DNA
attcttctatggtgctggtggaagtggg

SEQ ID NO: 26372 - DNA, 28 bp, synthetic construct
  source 1..28: mol_type = other DNA
tattcttctatggtgctggtggaagtgg

SEQ ID NO: 26373 - DNA, 28 bp, synthetic construct
  source 1..28: mol_type = other DNA
cagaattattcttctatggtgctggtgg

SEQ ID NO: 26374 - DNA, 28 bp, synthetic construct
  source 1..28: mol_type = other DNA
caccagcaccatagaagaataattctgg

SEQ ID NO: 26375 - DNA, 28 bp, synthetic construct
  source 1..28: mol_type = other DNA
accagcaccatagaagaataattctggg

SEQ ID NO: 26376 - DNA, 28 bp, synthetic construct
  source 1..28: mol_type = other DNA
gcccagaattattcttctatggtgctgg

SEQ ID NO: 26377 - DNA, 28 bp, synthetic construct
  source 1..28: mol_type = other DNA
acttctgcccagaattattcttctatgg

SEQ ID NO: 26378 - DNA, 28 bp, synthetic construct
  source 1..28: mol_type = other DNA
gaagtctgttttttttcatttttccagg

SEQ ID NO: 26379 - DNA, 28 bp, synthetic construct
  source 1..28: mol_type = other DNA
ttttttttcatttttccaggacagttgg

SEQ ID NO: 26380 - DNA, 28 bp, synthetic construct
  source 1..28: mol_type = other DNA
ttttccaggacagttggatattgtcagg

SEQ ID NO: 26381 - DNA, 28 bp, synthetic construct
  source 1..28: mol_type = other DNA
gtggcctgacaatatccaactgtcctgg

SEQ ID NO: 26382 - DNA, 28 bp, synthetic construct
  source 1..28: mol_type = other DNA
ctcactacatggctggggtcacaagtgg

SEQ ID NO: 26383 - DNA, 28 bp, synthetic construct
  source 1..28: mol_type = other DNA
cacttgtgaccccagccatgtagtgagg

SEQ ID NO: 26384 - DNA, 28 bp, synthetic construct
  source 1..28: mol_type = other DNA
acttgtgaccccagccatgtagtgaggg

SEQ ID NO: 26385 - DNA, 28 bp, synthetic construct
  source 1..28: mol_type = other DNA
aaagagcaccctcactacatggctgggg

SEQ ID NO: 26386 - DNA, 28 bp, synthetic construct
  source 1..28: mol_type = other DNA
gaaagagcaccctcactacatggctggg

SEQ ID NO: 26387 - DNA, 28 bp, synthetic construct
  source 1..28: mol_type = other DNA
agaaagagcaccctcactacatggctgg

SEQ ID NO: 26388 - DNA, 28 bp, synthetic construct
  source 1..28: mol_type = other DNA
acagagaaagagcaccctcactacatgg

SEQ ID NO: 26389 - DNA, 28 bp, synthetic construct
  source 1..28: mol_type = other DNA
ctgtgcctgctccttatgagtgcagtgg

SEQ ID NO: 26390 - DNA, 28 bp, synthetic construct
  source 1..28: mol_type = other DNA
gcctgctccttatgagtgcagtggaagg

SEQ ID NO: 26391 - DNA, 28 bp, synthetic construct
  source 1..28: mol_type = other DNA
tccttccactgcactcataaggagcagg

SEQ ID NO: 26392 - DNA, 28 bp, synthetic construct
  source 1..28: mol_type = other DNA
gtggcttccttccactgcactcataagg

SEQ ID NO: 26393 - DNA, 28 bp, synthetic construct
  source 1..28: mol_type = other DNA
agtgcagtggaaggaagccacacactgg

SEQ ID NO: 26394 - DNA, 28 bp, synthetic construct
  source 1..28: mol_type = other DNA
gccacacactggtcagtcatttcagagg

SEQ ID NO: 26395 - DNA, 28 bp, synthetic construct
  source 1..28: mol_type = other DNA
gcctctgaaatgactgaccagtgtgtgg

SEQ ID NO: 26396 - DNA, 28 bp, synthetic construct
  source 1..28: mol_type = other DNA
gtcatttcagaggcagcagatgcccagg

SEQ ID NO: 26397 - DNA, 28 bp, synthetic construct
  source 1..28: mol_type = other DNA
tcatttcagaggcagcagatgcccaggg

SEQ ID NO: 26398 - DNA, 28 bp, synthetic construct
  source 1..28: mol_type = other DNA
gcccagggagacccaagaaagagtcagg

SEQ ID NO: 26399 - DNA, 28 bp, synthetic construct
  source 1..28: mol_type = other DNA
acctgactctttcttgggtctccctggg

SEQ ID NO: 26400 - DNA, 28 bp, synthetic construct
  source 1..28: mol_type = other DNA
aacctgactctttcttgggtctccctgg

SEQ ID NO: 26401 - DNA, 28 bp, synthetic construct
  source 1..28: mol_type = other DNA
gggagacccaagaaagagtcaggttagg

SEQ ID NO: 26402 - DNA, 28 bp, synthetic construct
  source 1..28: mol_type = other DNA
ggagacccaagaaagagtcaggttaggg

SEQ ID NO: 26403 - DNA, 28 bp, synthetic construct
  source 1..28: mol_type = other DNA
ctgctccctaacctgactctttcttggg

SEQ ID NO: 26404 - DNA, 28 bp, synthetic construct
  source 1..28: mol_type = other DNA
actgctccctaacctgactctttcttgg

SEQ ID NO: 26405 - DNA, 28 bp, synthetic construct
  source 1..28: mol_type = other DNA
gtcaggttagggagcagtgaaagtgagg

SEQ ID NO: 26406 - DNA, 28 bp, synthetic construct
  source 1..28: mol_type = other DNA
aggttagggagcagtgaaagtgaggagg

SEQ ID NO: 26407 - DNA, 28 bp, synthetic construct
  source 1..28: mol_type = other DNA
ggttagggagcagtgaaagtgaggaggg

SEQ ID NO: 26408 - DNA, 28 bp, synthetic construct
  source 1..28: mol_type = other DNA
atttcttttaaaagttgtttaacgatgg

SEQ ID NO: 26409 - DNA, 28 bp, synthetic construct
  source 1..28: mol_type = other DNA
ttctatcgggcaaaacactagttggtgg

SEQ ID NO: 26410 - DNA, 28 bp, synthetic construct
  source 1..28: mol_type = other DNA
ctcttctatcgggcaaaacactagttgg

SEQ ID NO: 26411 - DNA, 28 bp, synthetic construct
  source 1..28: mol_type = other DNA
acgtgaacatgctggctcttctatcggg

SEQ ID NO: 26412 - DNA, 28 bp, synthetic construct
  source 1..28: mol_type = other DNA
aacgtgaacatgctggctcttctatcgg

SEQ ID NO: 26413 - DNA, 28 bp, synthetic construct
  source 1..28: mol_type = other DNA
cctaatttaaataacgtgaacatgctgg

SEQ ID NO: 26414 - DNA, 28 bp, synthetic construct
  source 1..28: mol_type = other DNA
gcatgttcacgttatttaaattaggtgg

SEQ ID NO: 26415 - DNA, 28 bp, synthetic construct
  source 1..28: mol_type = other DNA
atattgcatattcactttttcctttagg

SEQ ID NO: 26416 - DNA, 28 bp, synthetic construct
  source 1..28: mol_type = other DNA
ttggattgaaatcatctctacctaaagg

SEQ ID NO: 26417 - DNA, 28 bp, synthetic construct
  source 1..28: mol_type = other DNA
ggaaattttttaaagtaagagtatttgg

SEQ ID NO: 26418 - DNA, 28 bp, synthetic construct
  source 1..28: mol_type = other DNA
aatttcctttccccaagaatctccttgg

SEQ ID NO: 26419 - DNA, 28 bp, synthetic construct
  source 1..28: mol_type = other DNA
atttcctttccccaagaatctccttggg

SEQ ID NO: 26420 - DNA, 28 bp, synthetic construct
  source 1..28: mol_type = other DNA
aagtcccaaggagattcttggggaaagg

SEQ ID NO: 26421 - DNA, 28 bp, synthetic construct
  source 1..28: mol_type = other DNA
agtcaaagtcccaaggagattcttgggg

SEQ ID NO: 26422 - DNA, 28 bp, synthetic construct
  source 1..28: mol_type = other DNA
aagtcaaagtcccaaggagattcttggg

SEQ ID NO: 26423 - DNA, 28 bp, synthetic construct
  source 1..28: mol_type = other DNA
taagtcaaagtcccaaggagattcttgg

SEQ ID NO: 26424 - DNA, 28 bp, synthetic construct
  source 1..28: mol_type = other DNA
gctttaaaaataagtcaaagtcccaagg

SEQ ID NO: 26425 - DNA, 28 bp, synthetic construct
  source 1..28: mol_type = other DNA
ctttgacttatttttaaagctgtgttgg

SEQ ID NO: 26426 - DNA, 28 bp, synthetic construct
  source 1..28: mol_type = other DNA
gttccctgatgtgtctcgagcccattgg

SEQ ID NO: 26427 - DNA, 28 bp, synthetic construct
  source 1..28: mol_type = other DNA
ctaccaatgggctcgagacacatcaggg

SEQ ID NO: 26428 - DNA, 28 bp, synthetic construct
  source 1..28: mol_type = other DNA
cctaccaatgggctcgagacacatcagg

SEQ ID NO: 26429 - DNA, 28 bp, synthetic construct
  source 1..28: mol_type = other DNA
ctgatgtgtctcgagcccattggtaggg

SEQ ID NO: 26430 - DNA, 28 bp, synthetic construct
  source 1..28: mol_type = other DNA
gtgggctttgtatgaccctaccaatggg

SEQ ID NO: 26431 - DNA, 28 bp, synthetic construct
  source 1..28: mol_type = other DNA
cgtgggctttgtatgaccctaccaatgg

SEQ ID NO: 26432 - DNA, 28 bp, synthetic construct
  source 1..28: mol_type = other DNA
cattggtagggtcatacaaagcccacgg

SEQ ID NO: 26433 - DNA, 28 bp, synthetic construct
  source 1..28: mol_type = other DNA
atacaaagcccacggttacaagcagtgg

SEQ ID NO: 26434 - DNA, 28 bp, synthetic construct
  source 1..28: mol_type = other DNA
aaagcccacggttacaagcagtggtagg

SEQ ID NO: 26435 - DNA, 28 bp, synthetic construct
  source 1..28: mol_type = other DNA
caatcctaccactgcttgtaaccgtggg

SEQ ID NO: 26436 - DNA, 28 bp, synthetic construct
  source 1..28: mol_type = other DNA
gcaatcctaccactgcttgtaaccgtgg

SEQ ID NO: 26437 - DNA, 28 bp, synthetic construct
  source 1..28: mol_type = other DNA
acaagcagtggtaggattgcagccgtgg

SEQ ID NO: 26438 - DNA, 28 bp, synthetic construct
  source 1..28: mol_type = other DNA
caagcagtggtaggattgcagccgtggg

SEQ ID NO: 26439 - DNA, 28 bp, synthetic construct
  source 1..28: mol_type = other DNA
ggtaggattgcagccgtgggcctgctgg

SEQ ID NO: 26440 - DNA, 28 bp, synthetic construct
  source 1..28: mol_type = other DNA
tgtatgtgtgtgtccagcaggcccacgg

SEQ ID NO: 26441 - DNA, 28 bp, synthetic construct
  source 1..28: mol_type = other DNA
tctttggtgtatgtgtgtgtccagcagg

SEQ ID NO: 26442 - DNA, 28 bp, synthetic construct
  source 1..28: mol_type = other DNA
cacacacatacaccaaagatgtatttgg

SEQ ID NO: 26443 - DNA, 28 bp, synthetic construct
  source 1..28: mol_type = other DNA
catacaccaaagatgtatttggatctgg

SEQ ID NO: 26444 - DNA, 28 bp, synthetic construct
  source 1..28: mol_type = other DNA
atacaccaaagatgtatttggatctggg

SEQ ID NO: 26445 - DNA, 28 bp, synthetic construct
  source 1..28: mol_type = other DNA
gggtgcccagatccaaatacatctttgg

SEQ ID NO: 26446 - DNA, 28 bp, synthetic construct
  source 1..28: mol_type = other DNA
tatttggatctgggcaccccctcccagg

SEQ ID NO: 26447 - DNA, 28 bp, synthetic construct
  source 1..28: mol_type = other DNA
acgtgagtacagggatcctgggaggggg

SEQ ID NO: 26448 - DNA, 28 bp, synthetic construct
  source 1..28: mol_type = other DNA
cacgtgagtacagggatcctgggagggg

SEQ ID NO: 26449 - DNA, 28 bp, synthetic construct
  source 1..28: mol_type = other DNA
gcacgtgagtacagggatcctgggaggg

SEQ ID NO: 26450 - DNA, 28 bp, synthetic construct
  source 1..28: mol_type = other DNA
ggcacgtgagtacagggatcctgggagg

SEQ ID NO: 26451 - DNA, 28 bp, synthetic construct
  source 1..28: mol_type = other DNA
actggcacgtgagtacagggatcctggg

SEQ ID NO: 26452 - DNA, 28 bp, synthetic construct
  source 1..28: mol_type = other DNA
gactggcacgtgagtacagggatcctgg

SEQ ID NO: 26453 - DNA, 28 bp, synthetic construct
  source 1..28: mol_type = other DNA
gtcaggagactggcacgtgagtacaggg

SEQ ID NO: 26454 - DNA, 28 bp, synthetic construct
  source 1..28: mol_type = other DNA
agtcaggagactggcacgtgagtacagg

SEQ ID NO: 26455 - DNA, 28 bp, synthetic construct
  source 1..28: mol_type = other DNA
gagtaaagtgctctagtcaggagactgg

SEQ ID NO: 26456 - DNA, 28 bp, synthetic construct
  source 1..28: mol_type = other DNA
ggaaacagagtaaagtgctctagtcagg

SEQ ID NO: 26457 - DNA, 28 bp, synthetic construct
  source 1..28: mol_type = other DNA
tctgtttcctcagccctgcagcccctgg

SEQ ID NO: 26458 - DNA, 28 bp, synthetic construct
  source 1..28: mol_type = other DNA
ctgtttcctcagccctgcagcccctggg

SEQ ID NO: 26459 - DNA, 28 bp, synthetic construct
  source 1..28: mol_type = other DNA
tgtgctcccaggggctgcagggctgagg

SEQ ID NO: 26460 - DNA, 28 bp, synthetic construct
  source 1..28: mol_type = other DNA
ccctgcagcccctgggagcacacactgg

SEQ ID NO: 26461 - DNA, 28 bp, synthetic construct
  source 1..28: mol_type = other DNA
cctgcagcccctgggagcacacactggg

SEQ ID NO: 26462 - DNA, 28 bp, synthetic construct
  source 1..28: mol_type = other DNA
ggctgcacccagtgtgtgctcccagggg

SEQ ID NO: 26463 - DNA, 28 bp, synthetic construct
  source 1..28: mol_type = other DNA
gggctgcacccagtgtgtgctcccaggg

SEQ ID NO: 26464 - DNA, 28 bp, synthetic construct
  source 1..28: mol_type = other DNA
agggctgcacccagtgtgtgctcccagg

SEQ ID NO: 26465 - DNA, 28 bp, synthetic construct
  source 1..28: mol_type = other DNA
tgggagcacacactgggtgcagccctgg

SEQ ID NO: 26466 - DNA, 28 bp, synthetic construct
  source 1..28: mol_type = other DNA
gggagcacacactgggtgcagccctggg

SEQ ID NO: 26467 - DNA, 28 bp, synthetic construct
  source 1..28: mol_type = other DNA
cacacactgggtgcagccctgggccagg

SEQ ID NO: 26468 - DNA, 28 bp, synthetic construct
  source 1..28: mol_type = other DNA
actgggtgcagccctgggccaggcacgg

SEQ ID NO: 26469 - DNA, 28 bp, synthetic construct
  source 1..28: mol_type = other DNA
ctgggtgcagccctgggccaggcacggg

SEQ ID NO: 26470 - DNA, 28 bp, synthetic construct
  source 1..28: mol_type = other DNA
ggtgcagccctgggccaggcacgggagg

SEQ ID NO: 26471 - DNA, 28 bp, synthetic construct
  source 1..28: mol_type = other DNA
ggcagggcctcccgtgcctggcccaggg

SEQ ID NO: 26472 - DNA, 28 bp, synthetic construct
  source 1..28: mol_type = other DNA
gggcagggcctcccgtgcctggcccagg

SEQ ID NO: 26473 - DNA, 28 bp, synthetic construct
  source 1..28: mol_type = other DNA
agcacagggcagggcctcccgtgcctgg

SEQ ID NO: 26474 - DNA, 28 bp, synthetic construct
  source 1..28: mol_type = other DNA
cgggaggccctgccctgtgctgcccagg

SEQ ID NO: 26475 - DNA, 28 bp, synthetic construct
  source 1..28: mol_type = other DNA
gggaggccctgccctgtgctgcccaggg

SEQ ID NO: 26476 - DNA, 28 bp, synthetic construct
  source 1..28: mol_type = other DNA
ggaggccctgccctgtgctgcccagggg

SEQ ID NO: 26477 - DNA, 28 bp, synthetic construct
  source 1..28: mol_type = other DNA
cacagcccctgggcagcacagggcaggg

SEQ ID NO: 26478 - DNA, 28 bp, synthetic construct
  source 1..28: mol_type = other DNA
acacagcccctgggcagcacagggcagg

SEQ ID NO: 26479 - DNA, 28 bp, synthetic construct
  source 1..28: mol_type = other DNA
gtgcacacagcccctgggcagcacaggg

SEQ ID NO: 26480 - DNA, 28 bp, synthetic construct
  source 1..28: mol_type = other DNA
ggtgcacacagcccctgggcagcacagg

SEQ ID NO: 26481 - DNA, 28 bp, synthetic construct
  source 1..28: mol_type = other DNA
tgctcatgtggtgcacacagcccctggg

SEQ ID NO: 26482 - DNA, 28 bp, synthetic construct
  source 1..28: mol_type = other DNA
gtgctcatgtggtgcacacagcccctgg

SEQ ID NO: 26483 - DNA, 28 bp, synthetic construct
  source 1..28: mol_type = other DNA
tgcaccacatgagcacatttccctctgg

SEQ ID NO: 26484 - DNA, 28 bp, synthetic construct
  source 1..28: mol_type = other DNA
caggccagagggaaatgtgctcatgtgg

SEQ ID NO: 26485 - DNA, 28 bp, synthetic construct
  source 1..28: mol_type = other DNA
cacatgagcacatttccctctggcctgg

SEQ ID NO: 26486 - DNA, 28 bp, synthetic construct
  source 1..28: mol_type = other DNA
atgagcacatttccctctggcctggcgg

SEQ ID NO: 26487 - DNA, 28 bp, synthetic construct
  source 1..28: mol_type = other DNA
atttccctctggcctggcggcctccagg

SEQ ID NO: 26488 - DNA, 28 bp, synthetic construct
  source 1..28: mol_type = other DNA
ccctctggcctggcggcctccaggctgg

SEQ ID NO: 26489 - DNA, 28 bp, synthetic construct
  source 1..28: mol_type = other DNA
gccagcctggaggccgccaggccagagg

SEQ ID NO: 26490 - DNA, 28 bp, synthetic construct
  source 1..28: mol_type = other DNA
ggcctggcggcctccaggctggctgtgg

SEQ ID NO: 26491 - DNA, 28 bp, synthetic construct
  source 1..28: mol_type = other DNA
ttccacagccagcctggaggccgccagg

SEQ ID NO: 26492 - DNA, 28 bp, synthetic construct
  source 1..28: mol_type = other DNA
ggaactgtttccacagccagcctggagg

SEQ ID NO: 26493 - DNA, 28 bp, synthetic construct
  source 1..28: mol_type = other DNA
tcaggaactgtttccacagccagcctgg

SEQ ID NO: 26494 - DNA, 28 bp, synthetic construct
  source 1..28: mol_type = other DNA
aggctggctgtggaaacagttcctgagg

SEQ ID NO: 26495 - DNA, 28 bp, synthetic construct
  source 1..28: mol_type = other DNA
aattcatagaatctctaatttcctcagg

SEQ ID NO: 26496 - DNA, 28 bp, synthetic construct
  source 1..28: mol_type = other DNA
ggaaattagagattctatgaattgtagg

SEQ ID NO: 26497 - DNA, 28 bp, synthetic construct
  source 1..28: mol_type = other DNA
atgaattgtaggagtattaaagaccagg

SEQ ID NO: 26498 - DNA, 28 bp, synthetic construct
  source 1..28: mol_type = other DNA
gtaggagtattaaagaccaggctgttgg

SEQ ID NO: 26499 - DNA, 28 bp, synthetic construct
  source 1..28: mol_type = other DNA
gctttaagttctggtgccaacagcctgg

SEQ ID NO: 26500 - DNA, 28 bp, synthetic construct
  source 1..28: mol_type = other DNA
tggcaccagaacttaaagcgatgactgg

SEQ ID NO: 26501 - DNA, 28 bp, synthetic construct
  source 1..28: mol_type = other DNA
gacatccagtcatcgctttaagttctgg

SEQ ID NO: 26502 - DNA, 28 bp, synthetic construct
  source 1..28: mol_type = other DNA
tggatgtctctgtactgtatgtatctgg

SEQ ID NO: 26503 - DNA, 28 bp, synthetic construct
  source 1..28: mol_type = other DNA
cacgggaggcatactttctgcacagagg

SEQ ID NO: 26504 - DNA, 28 bp, synthetic construct
  source 1..28: mol_type = other DNA
ctctgtgcagaaagtatgcctcccgtgg

SEQ ID NO: 26505 - DNA, 28 bp, synthetic construct
  source 1..28: mol_type = other DNA
tctgtgcagaaagtatgcctcccgtggg

SEQ ID NO: 26506 - DNA, 28 bp, synthetic construct
  source 1..28: mol_type = other DNA
aaaggtaaaaacgtatacccacgggagg

SEQ ID NO: 26507 - DNA, 28 bp, synthetic construct
  source 1..28: mol_type = other DNA
aaaaaaggtaaaaacgtatacccacggg

SEQ ID NO: 26508 - DNA, 28 bp, synthetic construct
  source 1..28: mol_type = other DNA
taaaaaaggtaaaaacgtatacccacgg

SEQ ID NO: 26509 - DNA, 28 bp, synthetic construct
  source 1..28: mol_type = other DNA
tttctacaaaaatgttttttaaaaaagg

SEQ ID NO: 26510 - DNA, 28 bp, synthetic construct
  source 1..28: mol_type = other DNA
agaaaaaataattaaatcccctttttgg

SEQ ID NO: 26511 - DNA, 28 bp, synthetic construct
  source 1..28: mol_type = other DNA
aatcccctttttggaaacttactgcagg

SEQ ID NO: 26512 - DNA, 28 bp, synthetic construct
  source 1..28: mol_type = other DNA
aaacctgcagtaagtttccaaaaagggg

SEQ ID NO: 26513 - DNA, 28 bp, synthetic construct
  source 1..28: mol_type = other DNA
aaaacctgcagtaagtttccaaaaaggg

SEQ ID NO: 26514 - DNA, 28 bp, synthetic construct
  source 1..28: mol_type = other DNA
caaaacctgcagtaagtttccaaaaagg

SEQ ID NO: 26515 - DNA, 28 bp, synthetic construct
  source 1..28: mol_type = other DNA
tgccttgacaacctctccctatgtgagg

SEQ ID NO: 26516 - DNA, 28 bp, synthetic construct
  source 1..28: mol_type = other DNA
aacctcacatagggagaggttgtcaagg

SEQ ID NO: 26517 - DNA, 28 bp, synthetic construct
  source 1..28: mol_type = other DNA
ctttttacaaacctcacatagggagagg

SEQ ID NO: 26518 - DNA, 28 bp, synthetic construct
  source 1..28: mol_type = other DNA
ggacactttttacaaacctcacataggg

SEQ ID NO: 26519 - DNA, 28 bp, synthetic construct
  source 1..28: mol_type = other DNA
aggacactttttacaaacctcacatagg

SEQ ID NO: 26520 - DNA, 28 bp, synthetic construct
  source 1..28: mol_type = other DNA
ttattgcgtttctgtgttaagtcacagg

SEQ ID NO: 26521 - DNA, 28 bp, synthetic construct
  source 1..28: mol_type = other DNA
tgattcttcagatgcccttcccaactgg

SEQ ID NO: 26522 - DNA, 28 bp, synthetic construct
  source 1..28: mol_type = other DNA
tcttgatcaactaaccagttgggaaggg

SEQ ID NO: 26523 - DNA, 28 bp, synthetic construct
  source 1..28: mol_type = other DNA
ttcttgatcaactaaccagttgggaagg

SEQ ID NO: 26524 - DNA, 28 bp, synthetic construct
  source 1..28: mol_type = other DNA
aaaattcttgatcaactaaccagttggg

SEQ ID NO: 26525 - DNA, 28 bp, synthetic construct
  source 1..28: mol_type = other DNA
caaaattcttgatcaactaaccagttgg

SEQ ID NO: 26526 - DNA, 28 bp, synthetic construct
  source 1..28: mol_type = other DNA
caactggttagttgatcaagaattttgg

SEQ ID NO: 26527 - DNA, 28 bp, synthetic construct
  source 1..28: mol_type = other DNA
aactggttagttgatcaagaattttggg

SEQ ID NO: 26528 - DNA, 28 bp, synthetic construct
  source 1..28: mol_type = other DNA
actggttagttgatcaagaattttgggg

SEQ ID NO: 26529 - DNA, 28 bp, synthetic construct
  source 1..28: mol_type = other DNA
ctggttagttgatcaagaattttggggg

SEQ ID NO: 26530 - DNA, 28 bp, synthetic construct
  source 1..28: mol_type = other DNA
gttagttgatcaagaattttgggggtgg

SEQ ID NO: 26531 - DNA, 28 bp, synthetic construct
  source 1..28: mol_type = other DNA
ttagttgatcaagaattttgggggtggg

SEQ ID NO: 26532 - DNA, 28 bp, synthetic construct
  source 1..28: mol_type = other DNA
tagttgatcaagaattttgggggtgggg

SEQ ID NO: 26533 - DNA, 28 bp, synthetic construct
  source 1..28: mol_type = other DNA
agttgatcaagaattttgggggtggggg

SEQ ID NO: 26534 - DNA, 28 bp, synthetic construct
  source 1..28: mol_type = other DNA
tcaagaattttgggggtgggggttgcgg

SEQ ID NO: 26535 - DNA, 28 bp, synthetic construct
  source 1..28: mol_type = other DNA
attccttctgattaaaaaaatatagtgg

SEQ ID NO: 26536 - DNA, 28 bp, synthetic construct
  source 1..28: mol_type = other DNA
attccactatatttttttaatcagaagg

SEQ ID NO: 26537 - DNA, 28 bp, synthetic construct
  source 1..28: mol_type = other DNA
caatatatacattaagaaggggaaacgg

SEQ ID NO: 26538 - DNA, 28 bp, synthetic construct
  source 1..28: mol_type = other DNA
tactcacaatatatacattaagaagggg

SEQ ID NO: 26539 - DNA, 28 bp, synthetic construct
  source 1..28: mol_type = other DNA
atactcacaatatatacattaagaaggg

SEQ ID NO: 26540 - DNA, 28 bp, synthetic construct
  source 1..28: mol_type = other DNA
aatactcacaatatatacattaagaagg

SEQ ID NO: 26541 - DNA, 28 bp, synthetic construct
  source 1..28: mol_type = other DNA
tattgtgagtatttattagattcgtagg

SEQ ID NO: 26542 - DNA, 28 bp, synthetic construct
  source 1..28: mol_type = other DNA
ggaaacacaattgcacacagacatttgg

SEQ ID NO: 26543 - DNA, 28 bp, synthetic construct
  source 1..28: mol_type = other DNA
tgctgtacaaaattttacaaggtaaagg

SEQ ID NO: 26544 - DNA, 28 bp, synthetic construct
  source 1..28: mol_type = other DNA
tatttatgctgtacaaaattttacaagg

SEQ ID NO: 26545 - DNA, 28 bp, synthetic construct
  source 1..28: mol_type = other DNA
gtttttctcaactttttcaaaatcaagg

SEQ ID NO: 26546 - DNA, 28 bp, synthetic construct
  source 1..28: mol_type = other DNA
acaagttacagcattatgaaacagtagg

SEQ ID NO: 26547 - DNA, 28 bp, synthetic construct
  source 1..28: mol_type = other DNA
tgggacggcaggggagtgggagacaggg

SEQ ID NO: 26548 - DNA, 28 bp, synthetic construct
  source 1..28: mol_type = other DNA
atgggacggcaggggagtgggagacagg

SEQ ID NO: 26549 - DNA, 28 bp, synthetic construct
  source 1..28: mol_type = other DNA
taacttcatgggacggcaggggagtggg

SEQ ID NO: 26550 - DNA, 28 bp, synthetic construct
  source 1..28: mol_type = other DNA
ttaacttcatgggacggcaggggagtgg

SEQ ID NO: 26551 - DNA, 28 bp, synthetic construct
  source 1..28: mol_type = other DNA
aggagttaacttcatgggacggcagggg

SEQ ID NO: 26552 - DNA, 28 bp, synthetic construct
  source 1..28: mol_type = other DNA
caggagttaacttcatgggacggcaggg

SEQ ID NO: 26553 - DNA, 28 bp, synthetic construct
  source 1..28: mol_type = other DNA
tcaggagttaacttcatgggacggcagg

SEQ ID NO: 26554 - DNA, 28 bp, synthetic construct
  source 1..28: mol_type = other DNA
actctcaggagttaacttcatgggacgg

SEQ ID NO: 26555 - DNA, 28 bp, synthetic construct
  source 1..28: mol_type = other DNA
gacaactctcaggagttaacttcatggg

SEQ ID NO: 26556 - DNA, 28 bp, synthetic construct
  source 1..28: mol_type = other DNA
cgacaactctcaggagttaacttcatgg

SEQ ID NO: 26557 - DNA, 28 bp, synthetic construct
  source 1..28: mol_type = other DNA
catgaagttaactcctgagagttgtcgg

SEQ ID NO: 26558 - DNA, 28 bp, synthetic construct
  source 1..28: mol_type = other DNA
atgaagttaactcctgagagttgtcggg

SEQ ID NO: 26559 - DNA, 28 bp, synthetic construct
  source 1..28: mol_type = other DNA
tgaagttaactcctgagagttgtcgggg

SEQ ID NO: 26560 - DNA, 28 bp, synthetic construct
  source 1..28: mol_type = other DNA
gaagttaactcctgagagttgtcggggg

SEQ ID NO: 26561 - DNA, 28 bp, synthetic construct
  source 1..28: mol_type = other DNA
actcctgagagttgtcgggggtgactgg

SEQ ID NO: 26562 - DNA, 28 bp, synthetic construct
  source 1..28: mol_type = other DNA
tctccagtcacccccgacaactctcagg

SEQ ID NO: 26563 - DNA, 28 bp, synthetic construct
  source 1..28: mol_type = other DNA
actggagagctcattgcagaccacgtgg

SEQ ID NO: 26564 - DNA, 28 bp, synthetic construct
  source 1..28: mol_type = other DNA
ctcattgcagaccacgtggtcctccagg

SEQ ID NO: 26565 - DNA, 28 bp, synthetic construct
  source 1..28: mol_type = other DNA
tcattgcagaccacgtggtcctccaggg

SEQ ID NO: 26566 - DNA, 28 bp, synthetic construct
  source 1..28: mol_type = other DNA
ttgcagaccacgtggtcctccagggtgg

SEQ ID NO: 26567 - DNA, 28 bp, synthetic construct
  source 1..28: mol_type = other DNA
tggagagccaccctggaggaccacgtgg

SEQ ID NO: 26568 - DNA, 28 bp, synthetic construct
  source 1..28: mol_type = other DNA
gtcctccagggtggctctccaccttcgg

SEQ ID NO: 26569 - DNA, 28 bp, synthetic construct
  source 1..28: mol_type = other DNA
tcctccagggtggctctccaccttcggg

SEQ ID NO: 26570 - DNA, 28 bp, synthetic construct
  source 1..28: mol_type = other DNA
acccgaaggtggagagccaccctggagg

SEQ ID NO: 26571 - DNA, 28 bp, synthetic construct
  source 1..28: mol_type = other DNA
aggacccgaaggtggagagccaccctgg

SEQ ID NO: 26572 - DNA, 28 bp, synthetic construct
  source 1..28: mol_type = other DNA
agggtggctctccaccttcgggtcctgg

SEQ ID NO: 26573 - DNA, 28 bp, synthetic construct
  source 1..28: mol_type = other DNA
gactggaaataccaggacccgaaggtgg

SEQ ID NO: 26574 - DNA, 28 bp, synthetic construct
  source 1..28: mol_type = other DNA
cttgactggaaataccaggacccgaagg

SEQ ID NO: 26575 - DNA, 28 bp, synthetic construct
  source 1..28: mol_type = other DNA
tcgggtcctggtatttccagtcaagtgg

SEQ ID NO: 26576 - DNA, 28 bp, synthetic construct
  source 1..28: mol_type = other DNA
cgggtcctggtatttccagtcaagtggg

SEQ ID NO: 26577 - DNA, 28 bp, synthetic construct
  source 1..28: mol_type = other DNA
tgaaacccacttgactggaaataccagg

SEQ ID NO: 26578 - DNA, 28 bp, synthetic construct
  source 1..28: mol_type = other DNA
ttccagtcaagtgggtttcaattcttgg

SEQ ID NO: 26579 - DNA, 28 bp, synthetic construct
  source 1..28: mol_type = other DNA
tccagtcaagtgggtttcaattcttggg

SEQ ID NO: 26580 - DNA, 28 bp, synthetic construct
  source 1..28: mol_type = other DNA
gcccaagaattgaaacccacttgactgg

SEQ ID NO: 26581 - DNA, 28 bp, synthetic construct
  source 1..28: mol_type = other DNA
tcaaacacacacttcatcataagggcgg

SEQ ID NO: 26582 - DNA, 28 bp, synthetic construct
  source 1..28: mol_type = other DNA
gcatcaaacacacacttcatcataaggg

SEQ ID NO: 26583 - DNA, 28 bp, synthetic construct
  source 1..28: mol_type = other DNA
ggcatcaaacacacacttcatcataagg

SEQ ID NO: 26584 - DNA, 28 bp, synthetic construct
  source 1..28: mol_type = other DNA
tttgatgccagtgagaaactcagtctgg

SEQ ID NO: 26585 - DNA, 28 bp, synthetic construct
  source 1..28: mol_type = other DNA
atgccagtgagaaactcagtctggcagg

SEQ ID NO: 26586 - DNA, 28 bp, synthetic construct
  source 1..28: mol_type = other DNA
tagcctgccagactgagtttctcactgg

SEQ ID NO: 26587 - DNA, 28 bp, synthetic construct
  source 1..28: mol_type = other DNA
aaacagaaggttgctgggtatttcttgg

SEQ ID NO: 26588 - DNA, 28 bp, synthetic construct
  source 1..28: mol_type = other DNA
gctttggaacaaacagaaggttgctggg

SEQ ID NO: 26589 - DNA, 28 bp, synthetic construct
  source 1..28: mol_type = other DNA
tgctttggaacaaacagaaggttgctgg

SEQ ID NO: 26590 - DNA, 28 bp, synthetic construct
  source 1..28: mol_type = other DNA
agctagttgctttggaacaaacagaagg

SEQ ID NO: 26591 - DNA, 28 bp, synthetic construct
  source 1..28: mol_type = other DNA
tgcttgcatgataagctagttgctttgg

SEQ ID NO: 26592 - DNA, 28 bp, synthetic construct
  source 1..28: mol_type = other DNA
catgcaagcaaattttgctgactccagg

SEQ ID NO: 26593 - DNA, 28 bp, synthetic construct
  source 1..28: mol_type = other DNA
tttgctgactccaggctttatctttagg

SEQ ID NO: 26594 - DNA, 28 bp, synthetic construct
  source 1..28: mol_type = other DNA
tttttgttttcctaaagataaagcctgg

SEQ ID NO: 26595 - DNA, 28 bp, synthetic construct
  source 1..28: mol_type = other DNA
acaaaaaaaccaaagtattatcagcagg

SEQ ID NO: 26596 - DNA, 28 bp, synthetic construct
  source 1..28: mol_type = other DNA
aaaaaaccaaagtattatcagcaggtgg

SEQ ID NO: 26597 - DNA, 28 bp, synthetic construct
  source 1..28: mol_type = other DNA
aaaaaccaaagtattatcagcaggtggg

SEQ ID NO: 26598 - DNA, 28 bp, synthetic construct
  source 1..28: mol_type = other DNA
tctttcccacctgctgataatactttgg

SEQ ID NO: 26599 - DNA, 28 bp, synthetic construct
  source 1..28: mol_type = other DNA
ttcttttctaaacgctgagttgtcaggg

SEQ ID NO: 26600 - DNA, 28 bp, synthetic construct
  source 1..28: mol_type = other DNA
tttcttttctaaacgctgagttgtcagg

SEQ ID NO: 26601 - DNA, 28 bp, synthetic construct
  source 1..28: mol_type = other DNA
aagaaataaaatgtgccacttccagagg

SEQ ID NO: 26602 - DNA, 28 bp, synthetic construct
  source 1..28: mol_type = other DNA
aactgcaatgcagcacctctggaagtgg

SEQ ID NO: 26603 - DNA, 28 bp, synthetic construct
  source 1..28: mol_type = other DNA
ctgaacaactgcaatgcagcacctctgg

SEQ ID NO: 26604 - DNA, 28 bp, synthetic construct
  source 1..28: mol_type = other DNA
cagaggtgctgcattgcagttgttcagg

SEQ ID NO: 26605 - DNA, 28 bp, synthetic construct
  source 1..28: mol_type = other DNA
agaggtgctgcattgcagttgttcaggg

SEQ ID NO: 26606 - DNA, 28 bp, synthetic construct
  source 1..28: mol_type = other DNA
tgctgcattgcagttgttcagggctagg

SEQ ID NO: 26607 - DNA, 28 bp, synthetic construct
  source 1..28: mol_type = other DNA
gctgcattgcagttgttcagggctaggg

SEQ ID NO: 26608 - DNA, 28 bp, synthetic construct
  source 1..28: mol_type = other DNA
attgcagttgttcagggctagggccagg

SEQ ID NO: 26609 - DNA, 28 bp, synthetic construct
  source 1..28: mol_type = other DNA
cagttgttcagggctagggccaggcagg

SEQ ID NO: 26610 - DNA, 28 bp, synthetic construct
  source 1..28: mol_type = other DNA
gctagggccaggcaggacaagtgaatgg

SEQ ID NO: 26611 - DNA, 28 bp, synthetic construct
  source 1..28: mol_type = other DNA
ctagggccaggcaggacaagtgaatggg

SEQ ID NO: 26612 - DNA, 28 bp, synthetic construct
  source 1..28: mol_type = other DNA
gggccaggcaggacaagtgaatgggtgg

SEQ ID NO: 26613 - DNA, 28 bp, synthetic construct
  source 1..28: mol_type = other DNA
ggccaggcaggacaagtgaatgggtggg

SEQ ID NO: 26614 - DNA, 28 bp, synthetic construct
  source 1..28: mol_type = other DNA
gtcccacccattcacttgtcctgcctgg

SEQ ID NO: 26615 - DNA, 28 bp, synthetic construct
  source 1..28: mol_type = other DNA
ggcaggacaagtgaatgggtgggacagg

SEQ ID NO: 26616 - DNA, 28 bp, synthetic construct
  source 1..28: mol_type = other DNA
aggacaagtgaatgggtgggacaggtgg

SEQ ID NO: 26617 - DNA, 28 bp, synthetic construct
  source 1..28: mol_type = other DNA
gggtgggacaggtggctcctgcctaagg

SEQ ID NO: 26618 - DNA, 28 bp, synthetic construct
  source 1..28: mol_type = other DNA
gtggctcctgcctaaggaccacctcagg

SEQ ID NO: 26619 - DNA, 28 bp, synthetic construct
  source 1..28: mol_type = other DNA
tagtggcctgaggtggtccttaggcagg

SEQ ID NO: 26620 - DNA, 28 bp, synthetic construct
  source 1..28: mol_type = other DNA
gggttagtggcctgaggtggtccttagg

SEQ ID NO: 26621 - DNA, 28 bp, synthetic construct
  source 1..28: mol_type = other DNA
accacctcaggccactaaccccttgtgg

SEQ ID NO: 26622 - DNA, 28 bp, synthetic construct
  source 1..28: mol_type = other DNA
tccacaaggggttagtggcctgaggtgg

SEQ ID NO: 26623 - DNA, 28 bp, synthetic construct
  source 1..28: mol_type = other DNA
ttgtccacaaggggttagtggcctgagg

SEQ ID NO: 26624 - DNA, 28 bp, synthetic construct
  source 1..28: mol_type = other DNA
ctcacagttgtccacaaggggttagtgg

SEQ ID NO: 26625 - DNA, 28 bp, synthetic construct
  source 1..28: mol_type = other DNA
ccccttgtggacaactgtgagtagctgg

SEQ ID NO: 26626 - DNA, 28 bp, synthetic construct
  source 1..28: mol_type = other DNA
cccagctactcacagttgtccacaaggg

SEQ ID NO: 26627 - DNA, 28 bp, synthetic construct
  source 1..28: mol_type = other DNA
acccagctactcacagttgtccacaagg

SEQ ID NO: 26628 - DNA, 28 bp, synthetic construct
  source 1..28: mol_type = other DNA
gcacaggaagttgcacagcaggtggggg

SEQ ID NO: 26629 - DNA, 28 bp, synthetic construct
  source 1..28: mol_type = other DNA
agcacaggaagttgcacagcaggtgggg

SEQ ID NO: 26630 - DNA, 28 bp, synthetic construct
  source 1..28: mol_type = other DNA
aagcacaggaagttgcacagcaggtggg

SEQ ID NO: 26631 - DNA, 28 bp, synthetic construct
  source 1..28: mol_type = other DNA
aaagcacaggaagttgcacagcaggtgg

SEQ ID NO: 26632 - DNA, 28 bp, synthetic construct
  source 1..28: mol_type = other DNA
ctcaaagcacaggaagttgcacagcagg

SEQ ID NO: 26633 - DNA, 28 bp, synthetic construct
  source 1..28: mol_type = other DNA
ctgctgtgcaacttcctgtgctttgagg

SEQ ID NO: 26634 - DNA, 28 bp, synthetic construct
  source 1..28: mol_type = other DNA
tgtgcaacttcctgtgctttgaggttgg

SEQ ID NO: 26635 - DNA, 28 bp, synthetic construct
  source 1..28: mol_type = other DNA
acaagttagtccaacctcaaagcacagg

SEQ ID NO: 26636 - DNA, 28 bp, synthetic construct
  source 1..28: mol_type = other DNA
tttgaggttggactaacttgtcttcagg

SEQ ID NO: 26637 - DNA, 28 bp, synthetic construct
  source 1..28: mol_type = other DNA
cagccctccccacgccccacccatacgg

SEQ ID NO: 26638 - DNA, 28 bp, synthetic construct
  source 1..28: mol_type = other DNA
tgaccgtatgggtggggcgtggggaggg

SEQ ID NO: 26639 - DNA, 28 bp, synthetic construct
  source 1..28: mol_type = other DNA
gtgaccgtatgggtggggcgtggggagg

SEQ ID NO: 26640 - DNA, 28 bp, synthetic construct
  source 1..28: mol_type = other DNA
gcagtgaccgtatgggtggggcgtgggg

SEQ ID NO: 26641 - DNA, 28 bp, synthetic construct
  source 1..28: mol_type = other DNA
tgcagtgaccgtatgggtggggcgtggg

SEQ ID NO: 26642 - DNA, 28 bp, synthetic construct
  source 1..28: mol_type = other DNA
atgcagtgaccgtatgggtggggcgtgg

SEQ ID NO: 26643 - DNA, 28 bp, synthetic construct
  source 1..28: mol_type = other DNA
gccccacccatacggtcactgcatttgg

SEQ ID NO: 26644 - DNA, 28 bp, synthetic construct
  source 1..28: mol_type = other DNA
accaaatgcagtgaccgtatgggtgggg

SEQ ID NO: 26645 - DNA, 28 bp, synthetic construct
  source 1..28: mol_type = other DNA
gaccaaatgcagtgaccgtatgggtggg

SEQ ID NO: 26646 - DNA, 28 bp, synthetic construct
  source 1..28: mol_type = other DNA
tgaccaaatgcagtgaccgtatgggtgg

SEQ ID NO: 26647 - DNA, 28 bp, synthetic construct
  source 1..28: mol_type = other DNA
ggctgaccaaatgcagtgaccgtatggg

SEQ ID NO: 26648 - DNA, 28 bp, synthetic construct
  source 1..28: mol_type = other DNA
aggctgaccaaatgcagtgaccgtatgg

SEQ ID NO: 26649 - DNA, 28 bp, synthetic construct
  source 1..28: mol_type = other DNA
ctgcatttggtcagcctgcttcttcagg

SEQ ID NO: 26650 - DNA, 28 bp, synthetic construct
  source 1..28: mol_type = other DNA
aaggagggcatcgacctgaagaagcagg

SEQ ID NO: 26651 - DNA, 28 bp, synthetic construct
  source 1..28: mol_type = other DNA
tgaaggagatggagtatcagaaggaggg

SEQ ID NO: 26652 - DNA, 28 bp, synthetic construct
  source 1..28: mol_type = other DNA
ctgaaggagatggagtatcagaaggagg

SEQ ID NO: 26653 - DNA, 28 bp, synthetic construct
  source 1..28: mol_type = other DNA
ctccttctgatactccatctccttcagg

SEQ ID NO: 26654 - DNA, 28 bp, synthetic construct
  source 1..28: mol_type = other DNA
tccttctgatactccatctccttcaggg

SEQ ID NO: 26655 - DNA, 28 bp, synthetic construct
  source 1..28: mol_type = other DNA
cccctgaaggagatggagtatcagaagg

SEQ ID NO: 26656 - DNA, 28 bp, synthetic construct
  source 1..28: mol_type = other DNA
tctgatactccatctccttcaggggagg

SEQ ID NO: 26657 - DNA, 28 bp, synthetic construct
  source 1..28: mol_type = other DNA
atactccatctccttcaggggaggttgg

SEQ ID NO: 26658 - DNA, 28 bp, synthetic construct
  source 1..28: mol_type = other DNA
tactccatctccttcaggggaggttggg

SEQ ID NO: 26659 - DNA, 28 bp, synthetic construct
  source 1..28: mol_type = other DNA
actccatctccttcaggggaggttgggg

SEQ ID NO: 26660 - DNA, 28 bp, synthetic construct
  source 1..28: mol_type = other DNA
gggccccaacctcccctgaaggagatgg

SEQ ID NO: 26661 - DNA, 28 bp, synthetic construct
  source 1..28: mol_type = other DNA
ccttcaggggaggttggggccccactgg

SEQ ID NO: 26662 - DNA, 28 bp, synthetic construct
  source 1..28: mol_type = other DNA
aggggaggttggggccccactggactgg

SEQ ID NO: 26663 - DNA, 28 bp, synthetic construct
  source 1..28: mol_type = other DNA
ggggaggttggggccccactggactggg

SEQ ID NO: 26664 - DNA, 28 bp, synthetic construct
  source 1..28: mol_type = other DNA
tcacatcttgacacccagtccagtgggg

SEQ ID NO: 26665 - DNA, 28 bp, synthetic construct
  source 1..28: mol_type = other DNA
ttcacatcttgacacccagtccagtggg

SEQ ID NO: 26666 - DNA, 28 bp, synthetic construct
  source 1..28: mol_type = other DNA
tttcacatcttgacacccagtccagtgg

SEQ ID NO: 26667 - DNA, 28 bp, synthetic construct
  source 1..28: mol_type = other DNA
ctgggtgtcaagatgtgaaagcttatgg

SEQ ID NO: 26668 - DNA, 28 bp, synthetic construct
  source 1..28: mol_type = other DNA
tgggtgtcaagatgtgaaagcttatggg

SEQ ID NO: 26669 - DNA, 28 bp, synthetic construct
  source 1..28: mol_type = other DNA
gatgtgaaagcttatgggagctttaagg

SEQ ID NO: 26670 - DNA, 28 bp, synthetic construct
  source 1..28: mol_type = other DNA
ttatgggagctttaaggagacttcatgg

SEQ ID NO: 26671 - DNA, 28 bp, synthetic construct
  source 1..28: mol_type = other DNA
tgggagctttaaggagacttcatggtgg

SEQ ID NO: 26672 - DNA, 28 bp, synthetic construct
  source 1..28: mol_type = other DNA
aggagacttcatggtggttccatgcagg

SEQ ID NO: 26673 - DNA, 28 bp, synthetic construct
  source 1..28: mol_type = other DNA
agacttcatggtggttccatgcaggtgg

SEQ ID NO: 26674 - DNA, 28 bp, synthetic construct
  source 1..28: mol_type = other DNA
agcagggatggcagaaccacctgcatgg

SEQ ID NO: 26675 - DNA, 28 bp, synthetic construct
  source 1..28: mol_type = other DNA
ttctgccatccctgctgatttagcctgg

SEQ ID NO: 26676 - DNA, 28 bp, synthetic construct
  source 1..28: mol_type = other DNA
aggcaccaggctaaatcagcagggatgg

SEQ ID NO: 26677 - DNA, 28 bp, synthetic construct
  source 1..28: mol_type = other DNA
acacaggcaccaggctaaatcagcaggg

SEQ ID NO: 26678 - DNA, 28 bp, synthetic construct
  source 1..28: mol_type = other DNA
cacacaggcaccaggctaaatcagcagg

SEQ ID NO: 26679 - DNA, 28 bp, synthetic construct
  source 1..28: mol_type = other DNA
acgtgagtggacacacacaggcaccagg

SEQ ID NO: 26680 - DNA, 28 bp, synthetic construct
  source 1..28: mol_type = other DNA
cacgtgtacgtgagtggacacacacagg

SEQ ID NO: 26681 - DNA, 28 bp, synthetic construct
  source 1..28: mol_type = other DNA
ctgtgtgtgtccactcacgtacacgtgg

SEQ ID NO: 26682 - DNA, 28 bp, synthetic construct
  source 1..28: mol_type = other DNA
tgtgtgtgtccactcacgtacacgtggg

SEQ ID NO: 26683 - DNA, 28 bp, synthetic construct
  source 1..28: mol_type = other DNA
gtgtgtgtccactcacgtacacgtgggg

SEQ ID NO: 26684 - DNA, 28 bp, synthetic construct
  source 1..28: mol_type = other DNA
tgtgtccactcacgtacacgtggggtgg

SEQ ID NO: 26685 - DNA, 28 bp, synthetic construct
  source 1..28: mol_type = other DNA
gtgtccactcacgtacacgtggggtggg

SEQ ID NO: 26686 - DNA, 28 bp, synthetic construct
  source 1..28: mol_type = other DNA
tgtccactcacgtacacgtggggtgggg

SEQ ID NO: 26687 - DNA, 28 bp, synthetic construct
  source 1..28: mol_type = other DNA
gtccactcacgtacacgtggggtggggg

SEQ ID NO: 26688 - DNA, 28 bp, synthetic construct
  source 1..28: mol_type = other DNA
ttcccccaccccacgtgtacgtgagtgg

SEQ ID NO: 26689 - DNA, 28 bp, synthetic construct
  source 1..28: mol_type = other DNA
tgtctacagatgacgctaaatcagttgg

SEQ ID NO: 26690 - DNA, 28 bp, synthetic construct
  source 1..28: mol_type = other DNA
gtctacagatgacgctaaatcagttggg

SEQ ID NO: 26691 - DNA, 28 bp, synthetic construct
  source 1..28: mol_type = other DNA
tctacagatgacgctaaatcagttgggg

SEQ ID NO: 26692 - DNA, 28 bp, synthetic construct
  source 1..28: mol_type = other DNA
gtcaagttacttaactgggagcttgagg

SEQ ID NO: 26693 - DNA, 28 bp, synthetic construct
  source 1..28: mol_type = other DNA
ataaaagtagtcaagttacttaactggg

SEQ ID NO: 26694 - DNA, 28 bp, synthetic construct
  source 1..28: mol_type = other DNA
aataaaagtagtcaagttacttaactgg

SEQ ID NO: 26695 - DNA, 28 bp, synthetic construct
  source 1..28: mol_type = other DNA
gttaagtaacttgactacttttatttgg

SEQ ID NO: 26696 - DNA, 28 bp, synthetic construct
  source 1..28: mol_type = other DNA
ttaagtaacttgactacttttatttggg

SEQ ID NO: 26697 - DNA, 28 bp, synthetic construct
  source 1..28: mol_type = other DNA
tacagtaactagtggtcacagaatctgg

SEQ ID NO: 26698 - DNA, 28 bp, synthetic construct
  source 1..28: mol_type = other DNA
tgatgagttctgatacagtaactagtgg

SEQ ID NO: 26699 - DNA, 28 bp, synthetic construct
  source 1..28: mol_type = other DNA
actagttactgtatcagaactcatcagg

SEQ ID NO: 26700 - DNA, 28 bp, synthetic construct
  source 1..28: mol_type = other DNA
tacccacttataaatagcactgatctgg

SEQ ID NO: 26701 - DNA, 28 bp, synthetic construct
  source 1..28: mol_type = other DNA
agccagatcagtgctatttataagtggg

SEQ ID NO: 26702 - DNA, 28 bp, synthetic construct
  source 1..28: mol_type = other DNA
cagccagatcagtgctatttataagtgg

SEQ ID NO: 26703 - DNA, 28 bp, synthetic construct
  source 1..28: mol_type = other DNA
ctgatccatcactaacctgttttctagg

SEQ ID NO: 26704 - DNA, 28 bp, synthetic construct
  source 1..28: mol_type = other DNA
tgggtcctagaaaacaggttagtgatgg

SEQ ID NO: 26705 - DNA, 28 bp, synthetic construct
  source 1..28: mol_type = other DNA
ctacatacgctgggtcctagaaaacagg

SEQ ID NO: 26706 - DNA, 28 bp, synthetic construct
  source 1..28: mol_type = other DNA
ctgcaatacaaatgctacatacgctggg

SEQ ID NO: 26707 - DNA, 28 bp, synthetic construct
  source 1..28: mol_type = other DNA
actgcaatacaaatgctacatacgctgg

SEQ ID NO: 26708 - DNA, 28 bp, synthetic construct
  source 1..28: mol_type = other DNA
tgtagcatttgtattgcagtttccctgg

SEQ ID NO: 26709 - DNA, 28 bp, synthetic construct
  source 1..28: mol_type = other DNA
atcagtgcaaaacacaagtaagccaggg

SEQ ID NO: 26710 - DNA, 28 bp, synthetic construct
  source 1..28: mol_type = other DNA
catcagtgcaaaacacaagtaagccagg

SEQ ID NO: 26711 - DNA, 28 bp, synthetic construct
  source 1..28: mol_type = other DNA
gtgttttgcactgatgaattttgacagg

SEQ ID NO: 26712 - DNA, 28 bp, synthetic construct
  source 1..28: mol_type = other DNA
tgttttgcactgatgaattttgacaggg

SEQ ID NO: 26713 - DNA, 28 bp, synthetic construct
  source 1..28: mol_type = other DNA
ttacagcagtattgcacaagtaaagtgg

SEQ ID NO: 26714 - DNA, 28 bp, synthetic construct
  source 1..28: mol_type = other DNA
ctgccaaaaagtataaaaatacagtagg

SEQ ID NO: 26715 - DNA, 28 bp, synthetic construct
  source 1..28: mol_type = other DNA
attcctactgtatttttatactttttgg

SEQ ID NO: 26716 - DNA, 28 bp, synthetic construct
  source 1..28: mol_type = other DNA
aaaaagtataaaaatacagtaggaatgg

SEQ ID NO: 26717 - DNA, 28 bp, synthetic construct
  source 1..28: mol_type = other DNA
gaaagatgtacaagaaataaattagggg

SEQ ID NO: 26718 - DNA, 28 bp, synthetic construct
  source 1..28: mol_type = other DNA
agaaagatgtacaagaaataaattaggg

SEQ ID NO: 26719 - DNA, 28 bp, synthetic construct
  source 1..28: mol_type = other DNA
tagaaagatgtacaagaaataaattagg

SEQ ID NO: 26720 - DNA, 28 bp, synthetic construct
  source 1..28: mol_type = other DNA
aaaaacacttaacacatccaattaaagg

SEQ ID NO: 26721 - DNA, 28 bp, synthetic construct
  source 1..28: mol_type = other DNA
cagaagactttgcagaacctttaattgg

SEQ ID NO: 26722 - DNA, 28 bp, synthetic construct
  source 1..28: mol_type = other DNA
ttaaaggttctgcaaagtcttctgctgg

SEQ ID NO: 26723 - DNA, 28 bp, synthetic construct
  source 1..28: mol_type = other DNA
aaggttctgcaaagtcttctgctggtgg

SEQ ID NO: 26724 - DNA, 28 bp, synthetic construct
  source 1..28: mol_type = other DNA
aggttctgcaaagtcttctgctggtggg

SEQ ID NO: 26725 - DNA, 28 bp, synthetic construct
  source 1..28: mol_type = other DNA
ctgctggtgggtgctcttcatcccctgg

SEQ ID NO: 26726 - DNA, 28 bp, synthetic construct
  source 1..28: mol_type = other DNA
tttacaaagtaaactttacatccagggg

SEQ ID NO: 26727 - DNA, 28 bp, synthetic construct
  source 1..28: mol_type = other DNA
gtttacaaagtaaactttacatccaggg

SEQ ID NO: 26728 - DNA, 28 bp, synthetic construct
  source 1..28: mol_type = other DNA
tgtttacaaagtaaactttacatccagg

SEQ ID NO: 26729 - DNA, 28 bp, synthetic construct
  source 1..28: mol_type = other DNA
tttactttgtaaacaaacaactgtgagg

SEQ ID NO: 26730 - DNA, 28 bp, synthetic construct
  source 1..28: mol_type = other DNA
aacaaacaactgtgaggcaatctagagg

SEQ ID NO: 26731 - DNA, 28 bp, synthetic construct
  source 1..28: mol_type = other DNA
acaaacaactgtgaggcaatctagaggg

SEQ ID NO: 26732 - DNA, 28 bp, synthetic construct
  source 1..28: mol_type = other DNA
ggttagcgagcctcactttagtttccgg

SEQ ID NO: 26733 - DNA, 28 bp, synthetic construct
  source 1..28: mol_type = other DNA
gcgagcctcactttagtttccggagtgg

SEQ ID NO: 26734 - DNA, 28 bp, synthetic construct
  source 1..28: mol_type = other DNA
cgagcctcactttagtttccggagtggg

SEQ ID NO: 26735 - DNA, 28 bp, synthetic construct
  source 1..28: mol_type = other DNA
gaagcccactccggaaactaaagtgagg

SEQ ID NO: 26736 - DNA, 28 bp, synthetic construct
  source 1..28: mol_type = other DNA
cactttagtttccggagtgggcttcagg

SEQ ID NO: 26737 - DNA, 28 bp, synthetic construct
  source 1..28: mol_type = other DNA
gcaaagcaagacctgaagcccactccgg

SEQ ID NO: 26738 - DNA, 28 bp, synthetic construct
  source 1..28: mol_type = other DNA
cttcaggtcttgctttgcacatcaatgg

SEQ ID NO: 26739 - DNA, 28 bp, synthetic construct
  source 1..28: mol_type = other DNA
agaatattctcaagtcatgaatattagg

SEQ ID NO: 26740 - DNA, 28 bp, synthetic construct
  source 1..28: mol_type = other DNA
atgaatattaggtgtctgtcaatcttgg

SEQ ID NO: 26741 - DNA, 28 bp, synthetic construct
  source 1..28: mol_type = other DNA
tagatgacttcttattttatgttttagg

SEQ ID NO: 26742 - DNA, 28 bp, synthetic construct
  source 1..28: mol_type = other DNA
gtgcatctatgttcgtctgtgtgtttgg

SEQ ID NO: 26743 - DNA, 28 bp, synthetic construct
  source 1..28: mol_type = other DNA
gaacatagatgcacacaaacataaaagg

SEQ ID NO: 26744 - DNA, 28 bp, synthetic construct
  source 1..28: mol_type = other DNA
taaaaggactaacaatgaactgaaaagg

SEQ ID NO: 26745 - DNA, 28 bp, synthetic construct
  source 1..28: mol_type = other DNA
tgaaagtatgaaagcaggatgtaggtgg

SEQ ID NO: 26746 - DNA, 28 bp, synthetic construct
  source 1..28: mol_type = other DNA
tgttgaaagtatgaaagcaggatgtagg

SEQ ID NO: 26747 - DNA, 28 bp, synthetic construct
  source 1..28: mol_type = other DNA
taaattatgttgaaagtatgaaagcagg

SEQ ID NO: 26748 - DNA, 28 bp, synthetic construct
  source 1..28: mol_type = other DNA
ctttcaacataatttaacacattcaagg

SEQ ID NO: 26749 - DNA, 28 bp, synthetic construct
  source 1..28: mol_type = other DNA
aattcaaaatatctatctataccaatgg

SEQ ID NO: 26750 - DNA, 28 bp, synthetic construct
  source 1..28: mol_type = other DNA
aaaaaaaaaaaagtttgaaaaccattgg

SEQ ID NO: 26751 - DNA, 28 bp, synthetic construct
  source 1..28: mol_type = other DNA
tgagacgaagtcttgctctgttgccagg

SEQ ID NO: 26752 - DNA, 28 bp, synthetic construct
  source 1..28: mol_type = other DNA
acgaagtcttgctctgttgccaggctgg

SEQ ID NO: 26753 - DNA, 28 bp, synthetic construct
  source 1..28: mol_type = other DNA
gctctgttgccaggctggagtgcagtgg

SEQ ID NO: 26754 - DNA, 28 bp, synthetic construct
  source 1..28: mol_type = other DNA
gagattgcaccactgcactccagcctgg

SEQ ID NO: 26755 - DNA, 28 bp, synthetic construct
  source 1..28: mol_type = other DNA
aggctggagtgcagtggtgcaatctcgg

SEQ ID NO: 26756 - DNA, 28 bp, synthetic construct
  source 1..28: mol_type = other DNA
tcggctcactgcaacctctgcctcccgg

SEQ ID NO: 26757 - DNA, 28 bp, synthetic construct
  source 1..28: mol_type = other DNA
cggctcactgcaacctctgcctcccggg

SEQ ID NO: 26758 - DNA, 28 bp, synthetic construct
  source 1..28: mol_type = other DNA
agaatcacttgaacccgggaggcagagg

SEQ ID NO: 26759 - DNA, 28 bp, synthetic construct
  source 1..28: mol_type = other DNA
ggcaggagaatcacttgaacccgggagg

SEQ ID NO: 26760 - DNA, 28 bp, synthetic construct
  source 1..28: mol_type = other DNA
taaggcaggagaatcacttgaacccggg

SEQ ID NO: 26761 - DNA, 28 bp, synthetic construct
  source 1..28: mol_type = other DNA
ctaaggcaggagaatcacttgaacccgg

SEQ ID NO: 26762 - DNA, 28 bp, synthetic construct
  source 1..28: mol_type = other DNA
gtgattctcctgccttagcctcccaagg

SEQ ID NO: 26763 - DNA, 28 bp, synthetic construct
  source 1..28: mol_type = other DNA
ctcctgccttagcctcccaaggagctgg

SEQ ID NO: 26764 - DNA, 28 bp, synthetic construct
  source 1..28: mol_type = other DNA
tcctgccttagcctcccaaggagctggg

SEQ ID NO: 26765 - DNA, 28 bp, synthetic construct
  source 1..28: mol_type = other DNA
tcccagctccttgggaggctaaggcagg

SEQ ID NO: 26766 - DNA, 28 bp, synthetic construct
  source 1..28: mol_type = other DNA
gtagtcccagctccttgggaggctaagg

SEQ ID NO: 26767 - DNA, 28 bp, synthetic construct
  source 1..28: mol_type = other DNA
tagcctcccaaggagctgggactacagg

SEQ ID NO: 26768 - DNA, 28 bp, synthetic construct
  source 1..28: mol_type = other DNA
atgcctgtagtcccagctccttgggagg

SEQ ID NO: 26769 - DNA, 28 bp, synthetic construct
  source 1..28: mol_type = other DNA
tgcatgcctgtagtcccagctccttggg

SEQ ID NO: 26770 - DNA, 28 bp, synthetic construct
  source 1..28: mol_type = other DNA
gtgcatgcctgtagtcccagctccttgg

SEQ ID NO: 26771 - DNA, 28 bp, synthetic construct
  source 1..28: mol_type = other DNA
aaatacaaaaattatctgggcgtggtgg

SEQ ID NO: 26772 - DNA, 28 bp, synthetic construct
  source 1..28: mol_type = other DNA
taaaaatacaaaaattatctgggcgtgg

SEQ ID NO: 26773 - DNA, 28 bp, synthetic construct
  source 1..28: mol_type = other DNA
tttactaaaaatacaaaaattatctggg

SEQ ID NO: 26774 - DNA, 28 bp, synthetic construct
  source 1..28: mol_type = other DNA
ctttactaaaaatacaaaaattatctgg

SEQ ID NO: 26775 - DNA, 28 bp, synthetic construct
  source 1..28: mol_type = other DNA
ataatttttgtatttttagtaaagaagg

SEQ ID NO: 26776 - DNA, 28 bp, synthetic construct
  source 1..28: mol_type = other DNA
taatttttgtatttttagtaaagaaggg

SEQ ID NO: 26777 - DNA, 28 bp, synthetic construct
  source 1..28: mol_type = other DNA
tagtaaagaagggatttcaccatgttgg

SEQ ID NO: 26778 - DNA, 28 bp, synthetic construct
  source 1..28: mol_type = other DNA
aagaagggatttcaccatgttggccagg

SEQ ID NO: 26779 - DNA, 28 bp, synthetic construct
  source 1..28: mol_type = other DNA
gagatggagactgtcctggccaacatgg

SEQ ID NO: 26780 - DNA, 28 bp, synthetic construct
  source 1..28: mol_type = other DNA
cgaggtcaagagatggagactgtcctgg

SEQ ID NO: 26781 - DNA, 28 bp, synthetic construct
  source 1..28: mol_type = other DNA
gcgggcggatcacgaggtcaagagatgg

SEQ ID NO: 26782 - DNA, 28 bp, synthetic construct
  source 1..28: mol_type = other DNA
tcttgacctcgtgatccgcccgccttgg

SEQ ID NO: 26783 - DNA, 28 bp, synthetic construct
  source 1..28: mol_type = other DNA
ggaaggccaaggcgggcggatcacgagg

SEQ ID NO: 26784 - DNA, 28 bp, synthetic construct
  source 1..28: mol_type = other DNA
cagcacttcggaaggccaaggcgggcgg

SEQ ID NO: 26785 - DNA, 28 bp, synthetic construct
  source 1..28: mol_type = other DNA
cgcccgccttggccttccgaagtgctgg

SEQ ID NO: 26786 - DNA, 28 bp, synthetic construct
  source 1..28: mol_type = other DNA
gcccgccttggccttccgaagtgctggg

SEQ ID NO: 26787 - DNA, 28 bp, synthetic construct
  source 1..28: mol_type = other DNA
tcccagcacttcggaaggccaaggcggg

SEQ ID NO: 26788 - DNA, 28 bp, synthetic construct
  source 1..28: mol_type = other DNA
atcccagcacttcggaaggccaaggcgg

SEQ ID NO: 26789 - DNA, 28 bp, synthetic construct
  source 1..28: mol_type = other DNA
gtaatcccagcacttcggaaggccaagg

SEQ ID NO: 26790 - DNA, 28 bp, synthetic construct
  source 1..28: mol_type = other DNA
acgcttgtaatcccagcacttcggaagg

SEQ ID NO: 26791 - DNA, 28 bp, synthetic construct
  source 1..28: mol_type = other DNA
gctcacgcttgtaatcccagcacttcgg

SEQ ID NO: 26792 - DNA, 28 bp, synthetic construct
  source 1..28: mol_type = other DNA
gattacaagcgtgagccaccacacccgg

SEQ ID NO: 26793 - DNA, 28 bp, synthetic construct
  source 1..28: mol_type = other DNA
aaaaaacagtttgggccgggtgtggtgg

SEQ ID NO: 26794 - DNA, 28 bp, synthetic construct
  source 1..28: mol_type = other DNA
caaaaaaaacagtttgggccgggtgtgg

SEQ ID NO: 26795 - DNA, 28 bp, synthetic construct
  source 1..28: mol_type = other DNA
acaaacaaaaaaaacagtttgggccggg

SEQ ID NO: 26796 - DNA, 28 bp, synthetic construct
  source 1..28: mol_type = other DNA
aacaaacaaaaaaaacagtttgggccgg

SEQ ID NO: 26797 - DNA, 28 bp, synthetic construct
  source 1..28: mol_type = other DNA
aagaaacaaacaaaaaaaacagtttggg

SEQ ID NO: 26798 - DNA, 28 bp, synthetic construct
  source 1..28: mol_type = other DNA
aaagaaacaaacaaaaaaaacagtttgg

SEQ ID NO: 26799 - DNA, 28 bp, synthetic construct
  source 1..28: mol_type = other DNA
ttttttttgtttgtttcttttgagatgg

SEQ ID NO: 26800 - DNA, 28 bp, synthetic construct
  source 1..28: mol_type = other DNA
gagatggagtctcgctctgtcgccctgg

SEQ ID NO: 26801 - DNA, 28 bp, synthetic construct
  source 1..28: mol_type = other DNA
tggagtctcgctctgtcgccctggctgg

SEQ ID NO: 26802 - DNA, 28 bp, synthetic construct
  source 1..28: mol_type = other DNA
agatcacgtcactgcactccagccaggg

SEQ ID NO: 26803 - DNA, 28 bp, synthetic construct
  source 1..28: mol_type = other DNA
gagatcacgtcactgcactccagccagg

SEQ ID NO: 26804 - DNA, 28 bp, synthetic construct
  source 1..28: mol_type = other DNA
tcagctcactgcaacctccatctcctgg

SEQ ID NO: 26805 - DNA, 28 bp, synthetic construct
  source 1..28: mol_type = other DNA
cagctcactgcaacctccatctcctggg

SEQ ID NO: 26806 - DNA, 28 bp, synthetic construct
  source 1..28: mol_type = other DNA
agaattgcttgaacccaggagatggagg

SEQ ID NO: 26807 - DNA, 28 bp, synthetic construct
  source 1..28: mol_type = other DNA
aggagaattgcttgaacccaggagatgg

SEQ ID NO: 26808 - DNA, 28 bp, synthetic construct
  source 1..28: mol_type = other DNA
tgaggtaggagaattgcttgaacccagg

SEQ ID NO: 26809 - DNA, 28 bp, synthetic construct
  source 1..28: mol_type = other DNA
tctcagctactcaggaggctgaggtagg

SEQ ID NO: 26810 - DNA, 28 bp, synthetic construct
  source 1..28: mol_type = other DNA
gtaatctcagctactcaggaggctgagg

SEQ ID NO: 26811 - DNA, 28 bp, synthetic construct
  source 1..28: mol_type = other DNA
cagcctcctgagtagctgagattacagg

SEQ ID NO: 26812 - DNA, 28 bp, synthetic construct
  source 1..28: mol_type = other DNA
gcacctgtaatctcagctactcaggagg

SEQ ID NO: 26813 - DNA, 28 bp, synthetic construct
  source 1..28: mol_type = other DNA
agggcacctgtaatctcagctactcagg

SEQ ID NO: 26814 - DNA, 28 bp, synthetic construct
  source 1..28: mol_type = other DNA
gcaaaaattagctgggcatggtggaggg

SEQ ID NO: 26815 - DNA, 28 bp, synthetic construct
  source 1..28: mol_type = other DNA
tgcaaaaattagctgggcatggtggagg

SEQ ID NO: 26816 - DNA, 28 bp, synthetic construct
  source 1..28: mol_type = other DNA
aaatgcaaaaattagctgggcatggtgg

SEQ ID NO: 26817 - DNA, 28 bp, synthetic construct
  source 1..28: mol_type = other DNA
taaaaatgcaaaaattagctgggcatgg

SEQ ID NO: 26818 - DNA, 28 bp, synthetic construct
  source 1..28: mol_type = other DNA
tctactaaaaatgcaaaaattagctggg

SEQ ID NO: 26819 - DNA, 28 bp, synthetic construct
  source 1..28: mol_type = other DNA
ctctactaaaaatgcaaaaattagctgg

SEQ ID NO: 26820 - DNA, 28 bp, synthetic construct
  source 1..28: mol_type = other DNA
ctaatttttgcatttttagtagagatgg

SEQ ID NO: 26821 - DNA, 28 bp, synthetic construct
  source 1..28: mol_type = other DNA
tagtagagatggtgtttcaccacgttgg

SEQ ID NO: 26822 - DNA, 28 bp, synthetic construct
  source 1..28: mol_type = other DNA
gagatggtgtttcaccacgttggccagg

SEQ ID NO: 26823 - DNA, 28 bp, synthetic construct
  source 1..28: mol_type = other DNA
tggtgtttcaccacgttggccaggctgg

SEQ ID NO: 26824 - DNA, 28 bp, synthetic construct
  source 1..28: mol_type = other DNA
gagttcaagaccagcctggccaacgtgg

SEQ ID NO: 26825 - DNA, 28 bp, synthetic construct
  source 1..28: mol_type = other DNA
tgaggtcaggagttcaagaccagcctgg

SEQ ID NO: 26826 - DNA, 28 bp, synthetic construct
  source 1..28: mol_type = other DNA
aggctggtcttgaactcctgacctcagg

SEQ ID NO: 26827 - DNA, 28 bp, synthetic construct
  source 1..28: mol_type = other DNA
tgaagtgggcagatcacctgaggtcagg

SEQ ID NO: 26828 - DNA, 28 bp, synthetic construct
  source 1..28: mol_type = other DNA
gaggctgaagtgggcagatcacctgagg

SEQ ID NO: 26829 - DNA, 28 bp, synthetic construct
  source 1..28: mol_type = other DNA
tgcccacttcagcctcccaaagtgctgg

SEQ ID NO: 26830 - DNA, 28 bp, synthetic construct
  source 1..28: mol_type = other DNA
gcccacttcagcctcccaaagtgctggg

SEQ ID NO: 26831 - DNA, 28 bp, synthetic construct
  source 1..28: mol_type = other DNA
tcccagcactttgggaggctgaagtggg

SEQ ID NO: 26832 - DNA, 28 bp, synthetic construct
  source 1..28: mol_type = other DNA
atcccagcactttgggaggctgaagtgg

SEQ ID NO: 26833 - DNA, 28 bp, synthetic construct
  source 1..28: mol_type = other DNA
cagcctcccaaagtgctgggattacagg

SEQ ID NO: 26834 - DNA, 28 bp, synthetic construct
  source 1..28: mol_type = other DNA
atgcctgtaatcccagcactttgggagg

SEQ ID NO: 26835 - DNA, 28 bp, synthetic construct
  source 1..28: mol_type = other DNA
ctcatgcctgtaatcccagcactttggg

SEQ ID NO: 26836 - DNA, 28 bp, synthetic construct
  source 1..28: mol_type = other DNA
gctcatgcctgtaatcccagcactttgg

SEQ ID NO: 26837 - DNA, 28 bp, synthetic construct
  source 1..28: mol_type = other DNA
ttaaaaacagtttggtcgggcgcggtgg

SEQ ID NO: 26838 - DNA, 28 bp, synthetic construct
  source 1..28: mol_type = other DNA
catttaaaaacagtttggtcgggcgcgg

SEQ ID NO: 26839 - DNA, 28 bp, synthetic construct
  source 1..28: mol_type = other DNA
gttatcatttaaaaacagtttggtcggg

SEQ ID NO: 26840 - DNA, 28 bp, synthetic construct
  source 1..28: mol_type = other DNA
agttatcatttaaaaacagtttggtcgg

SEQ ID NO: 26841 - DNA, 28 bp, synthetic construct
  source 1..28: mol_type = other DNA
gggcagttatcatttaaaaacagtttgg

SEQ ID NO: 26842 - DNA, 28 bp, synthetic construct
  source 1..28: mol_type = other DNA
gcataaggcttaagtattttaaaggggg

SEQ ID NO: 26843 - DNA, 28 bp, synthetic construct
  source 1..28: mol_type = other DNA
tgcataaggcttaagtattttaaagggg

SEQ ID NO: 26844 - DNA, 28 bp, synthetic construct
  source 1..28: mol_type = other DNA
ctgcataaggcttaagtattttaaaggg

SEQ ID NO: 26845 - DNA, 28 bp, synthetic construct
  source 1..28: mol_type = other DNA
tctgcataaggcttaagtattttaaagg

SEQ ID NO: 26846 - DNA, 28 bp, synthetic construct
  source 1..28: mol_type = other DNA
ttaagccttatgcagaaatcttatgtgg

SEQ ID NO: 26847 - DNA, 28 bp, synthetic construct
  source 1..28: mol_type = other DNA
atatgccacataagatttctgcataagg

SEQ ID NO: 26848 - DNA, 28 bp, synthetic construct
  source 1..28: mol_type = other DNA
atcttatgtggcatataaagagacaagg

SEQ ID NO: 26849 - DNA, 28 bp, synthetic construct
  source 1..28: mol_type = other DNA
ataaagagacaaggcagagatgctgtgg

SEQ ID NO: 26850 - DNA, 28 bp, synthetic construct
  source 1..28: mol_type = other DNA
gttgaaagtaacctcttgacccacctgg

SEQ ID NO: 26851 - DNA, 28 bp, synthetic construct
  source 1..28: mol_type = other DNA
tcattggatgtccaggtgggtcaagagg

SEQ ID NO: 26852 - DNA, 28 bp, synthetic construct
  source 1..28: mol_type = other DNA
aactatgctcattggatgtccaggtggg

SEQ ID NO: 26853 - DNA, 28 bp, synthetic construct
  source 1..28: mol_type = other DNA
aaactatgctcattggatgtccaggtgg

SEQ ID NO: 26854 - DNA, 28 bp, synthetic construct
  source 1..28: mol_type = other DNA
ttcaaactatgctcattggatgtccagg

SEQ ID NO: 26855 - DNA, 28 bp, synthetic construct
  source 1..28: mol_type = other DNA
tcagtggttttcaaactatgctcattgg

SEQ ID NO: 26856 - DNA, 28 bp, synthetic construct
  source 1..28: mol_type = other DNA
gcatagtttgaaaaccactgaaataagg

SEQ ID NO: 26857 - DNA, 28 bp, synthetic construct
  source 1..28: mol_type = other DNA
ttatggatagcataccttatttcagtgg

SEQ ID NO: 26858 - DNA, 28 bp, synthetic construct
  source 1..28: mol_type = other DNA
gaggcatggatagcatacattattatgg

SEQ ID NO: 26859 - DNA, 28 bp, synthetic construct
  source 1..28: mol_type = other DNA
ttacaaatttaattgctaggaggcatgg

SEQ ID NO: 26860 - DNA, 28 bp, synthetic construct
  source 1..28: mol_type = other DNA
tgttgttacaaatttaattgctaggagg

SEQ ID NO: 26861 - DNA, 28 bp, synthetic construct
  source 1..28: mol_type = other DNA
aattgttgttacaaatttaattgctagg

SEQ ID NO: 26862 - DNA, 28 bp, synthetic construct
  source 1..28: mol_type = other DNA
taagtaagacaaattaaacactgaatgg

SEQ ID NO: 26863 - DNA, 28 bp, synthetic construct
  source 1..28: mol_type = other DNA
acactgaatggaatgttgaaatctgagg

SEQ ID NO: 26864 - DNA, 28 bp, synthetic construct
  source 1..28: mol_type = other DNA
ttcattaagttaaaatgacaatgtaagg

SEQ ID NO: 26865 - DNA, 28 bp, synthetic construct
  source 1..28: mol_type = other DNA
atgtagttggggtagattatgatttagg

SEQ ID NO: 26866 - DNA, 28 bp, synthetic construct
  source 1..28: mol_type = other DNA
tttcatgaaaatttcaatgtagttgggg

SEQ ID NO: 26867 - DNA, 28 bp, synthetic construct
  source 1..28: mol_type = other DNA
ttttcatgaaaatttcaatgtagttggg

SEQ ID NO: 26868 - DNA, 28 bp, synthetic construct
  source 1..28: mol_type = other DNA
tttttcatgaaaatttcaatgtagttgg

SEQ ID NO: 26869 - DNA, 28 bp, synthetic construct
  source 1..28: mol_type = other DNA
tcatgaaaaataaacatatcaataatgg

SEQ ID NO: 26870 - DNA, 28 bp, synthetic construct
  source 1..28: mol_type = other DNA
catgaaaaataaacatatcaataatggg

SEQ ID NO: 26871 - DNA, 28 bp, synthetic construct
  source 1..28: mol_type = other DNA
gttggtcaagactttgtaaagaaattgg

SEQ ID NO: 26872 - DNA, 28 bp, synthetic construct
  source 1..28: mol_type = other DNA
ttactgggatagtcaggtaaacagttgg

SEQ ID NO: 26873 - DNA, 28 bp, synthetic construct
  source 1..28: mol_type = other DNA
aactgtttacctgactatcccagtaagg

SEQ ID NO: 26874 - DNA, 28 bp, synthetic construct
  source 1..28: mol_type = other DNA
gaaaattctccttactgggatagtcagg

SEQ ID NO: 26875 - DNA, 28 bp, synthetic construct
  source 1..28: mol_type = other DNA
tctttgaaggaaaattctccttactggg

SEQ ID NO: 26876 - DNA, 28 bp, synthetic construct
  source 1..28: mol_type = other DNA
atctttgaaggaaaattctccttactgg

SEQ ID NO: 26877 - DNA, 28 bp, synthetic construct
  source 1..28: mol_type = other DNA
agaattttccttcaaagatatttttagg

SEQ ID NO: 26878 - DNA, 28 bp, synthetic construct
  source 1..28: mol_type = other DNA
aagtttttcctaaaaatatctttgaagg

SEQ ID NO: 26879 - DNA, 28 bp, synthetic construct
  source 1..28: mol_type = other DNA
tctttgtttgcttttctttttaaaatgg

SEQ ID NO: 26880 - DNA, 28 bp, synthetic construct
  source 1..28: mol_type = other DNA
ctttgtttgcttttctttttaaaatggg

SEQ ID NO: 26881 - DNA, 28 bp, synthetic construct
  source 1..28: mol_type = other DNA
tttgtttgcttttctttttaaaatgggg

SEQ ID NO: 26882 - DNA, 28 bp, synthetic construct
  source 1..28: mol_type = other DNA
aagtttgatatgagcagttagaagttgg

SEQ ID NO: 26883 - DNA, 28 bp, synthetic construct
  source 1..28: mol_type = other DNA
catatcaaacttctctttagaaaaatgg

SEQ ID NO: 26884 - DNA, 28 bp, synthetic construct
  source 1..28: mol_type = other DNA
aaattgtatgtcgattgaattgtactgg

SEQ ID NO: 26885 - DNA, 28 bp, synthetic construct
  source 1..28: mol_type = other DNA
aacacttttattcttaagcatttcaggg

SEQ ID NO: 26886 - DNA, 28 bp, synthetic construct
  source 1..28: mol_type = other DNA
caacacttttattcttaagcatttcagg

SEQ ID NO: 26887 - DNA, 28 bp, synthetic construct
  source 1..28: mol_type = other DNA
gtaatgtataatgtactattgacatggg

SEQ ID NO: 26888 - DNA, 28 bp, synthetic construct
  source 1..28: mol_type = other DNA
tgtaatgtataatgtactattgacatgg

SEQ ID NO: 26889 - DNA, 28 bp, synthetic construct
  source 1..28: mol_type = other DNA
aatattgtggttttatctacgttattgg

SEQ ID NO: 26890 - DNA, 28 bp, synthetic construct
  source 1..28: mol_type = other DNA
cacttgatataagcaataaatattgtgg

SEQ ID NO: 26891 - DNA, 28 bp, synthetic construct
  source 1..28: mol_type = other DNA
aatatttattgcttatatcaagtgcagg

SEQ ID NO: 26892 - DNA, 28 bp, synthetic construct
  source 1..28: mol_type = other DNA
acaggatttgtttttggaggctatctgg

SEQ ID NO: 26893 - DNA, 28 bp, synthetic construct
  source 1..28: mol_type = other DNA
cctttatcacaggatttgtttttggagg

SEQ ID NO: 26894 - DNA, 28 bp, synthetic construct
  source 1..28: mol_type = other DNA
tatcctttatcacaggatttgtttttgg

SEQ ID NO: 26895 - DNA, 28 bp, synthetic construct
  source 1..28: mol_type = other DNA
ccaacattgagatatcctttatcacagg

SEQ ID NO: 26896 - DNA, 28 bp, synthetic construct
  source 1..28: mol_type = other DNA
gataaaggatatctcaatgttggtcagg

SEQ ID NO: 26897 - DNA, 28 bp, synthetic construct
  source 1..28: mol_type = other DNA
aaagacattcatgtttgttaaaaactgg

SEQ ID NO: 26898 - DNA, 28 bp, synthetic construct
  source 1..28: mol_type = other DNA
ttattttagacagccatttacagtttgg

SEQ ID NO: 26899 - DNA, 28 bp, synthetic construct
  source 1..28: mol_type = other DNA
tattttagacagccatttacagtttggg

SEQ ID NO: 26900 - DNA, 28 bp, synthetic construct
  source 1..28: mol_type = other DNA
attttagacagccatttacagtttgggg

SEQ ID NO: 26901 - DNA, 28 bp, synthetic construct
  source 1..28: mol_type = other DNA
cagccatttacagtttggggttcagagg

SEQ ID NO: 26902 - DNA, 28 bp, synthetic construct
  source 1..28: mol_type = other DNA
gttcctctgaaccccaaactgtaaatgg

SEQ ID NO: 26903 - DNA, 28 bp, synthetic construct
  source 1..28: mol_type = other DNA
cctgcagtcaagagtcctgagatgttgg

SEQ ID NO: 26904 - DNA, 28 bp, synthetic construct
  source 1..28: mol_type = other DNA
ctgcagtcaagagtcctgagatgttggg

SEQ ID NO: 26905 - DNA, 28 bp, synthetic construct
  source 1..28: mol_type = other DNA
tttacagtcacaagcccaacatctcagg

SEQ ID NO: 26906 - DNA, 28 bp, synthetic construct
  source 1..28: mol_type = other DNA
cttgtgactgtaaatatcacttatctgg

SEQ ID NO: 26907 - DNA, 28 bp, synthetic construct
  source 1..28: mol_type = other DNA
gatgtctattctactgcaccgtttttgg

SEQ ID NO: 26908 - DNA, 28 bp, synthetic construct
  source 1..28: mol_type = other DNA
atgtctattctactgcaccgtttttggg

SEQ ID NO: 26909 - DNA, 28 bp, synthetic construct
  source 1..28: mol_type = other DNA
tctactgcaccgtttttgggatatgagg

SEQ ID NO: 26910 - DNA, 28 bp, synthetic construct
  source 1..28: mol_type = other DNA
cagcaaacgcctcatatcccaaaaacgg

SEQ ID NO: 26911 - DNA, 28 bp, synthetic construct
  source 1..28: mol_type = other DNA
actgacagtgctacattaatcatagggg

SEQ ID NO: 26912 - DNA, 28 bp, synthetic construct
  source 1..28: mol_type = other DNA
aactgacagtgctacattaatcataggg

SEQ ID NO: 26913 - DNA, 28 bp, synthetic construct
  source 1..28: mol_type = other DNA
taactgacagtgctacattaatcatagg

SEQ ID NO: 26914 - DNA, 28 bp, synthetic construct
  source 1..28: mol_type = other DNA
gtcagttactagtgcagaagcttgctgg

SEQ ID NO: 26915 - DNA, 28 bp, synthetic construct
  source 1..28: mol_type = other DNA
tcagttactagtgcagaagcttgctggg

SEQ ID NO: 26916 - DNA, 28 bp, synthetic construct
  source 1..28: mol_type = other DNA
ttgctgggcaaaattaattgtttatagg

SEQ ID NO: 26917 - DNA, 28 bp, synthetic construct
  source 1..28: mol_type = other DNA
tgctgggcaaaattaattgtttataggg

SEQ ID NO: 26918 - DNA, 28 bp, synthetic construct
  source 1..28: mol_type = other DNA
cattttggttggcgcttttgttggctgg

SEQ ID NO: 26919 - DNA, 28 bp, synthetic construct
  source 1..28: mol_type = other DNA
cagtcattttggttggcgcttttgttgg

SEQ ID NO: 26920 - DNA, 28 bp, synthetic construct
  source 1..28: mol_type = other DNA
tggggtttatgtcagtcattttggttgg

SEQ ID NO: 26921 - DNA, 28 bp, synthetic construct
  source 1..28: mol_type = other DNA
aagatggggtttatgtcagtcattttgg

SEQ ID NO: 26922 - DNA, 28 bp, synthetic construct
  source 1..28: mol_type = other DNA
acataaaccccatcttagtgagaatagg

SEQ ID NO: 26923 - DNA, 28 bp, synthetic construct
  source 1..28: mol_type = other DNA
ttggcaacctattctcactaagatgggg

SEQ ID NO: 26924 - DNA, 28 bp, synthetic construct
  source 1..28: mol_type = other DNA
attggcaacctattctcactaagatggg

SEQ ID NO: 26925 - DNA, 28 bp, synthetic construct
  source 1..28: mol_type = other DNA
tattggcaacctattctcactaagatgg

SEQ ID NO: 26926 - DNA, 28 bp, synthetic construct
  source 1..28: mol_type = other DNA
acgaaaaagaaaaaggtggttatattgg

SEQ ID NO: 26927 - DNA, 28 bp, synthetic construct
  source 1..28: mol_type = other DNA
tgagaatgaacgaaaaagaaaaaggtgg

SEQ ID NO: 26928 - DNA, 28 bp, synthetic construct
  source 1..28: mol_type = other DNA
aaatgagaatgaacgaaaaagaaaaagg

SEQ ID NO: 26929 - DNA, 28 bp, synthetic construct
  source 1..28: mol_type = other DNA
aagtgaaaggaagtgcacacagagcagg

SEQ ID NO: 26930 - DNA, 28 bp, synthetic construct
  source 1..28: mol_type = other DNA
gcaggacttgagtactctaacacagagg

SEQ ID NO: 26931 - DNA, 28 bp, synthetic construct
  source 1..28: mol_type = other DNA
ttgagtactctaacacagaggacctagg

SEQ ID NO: 26932 - DNA, 28 bp, synthetic construct
  source 1..28: mol_type = other DNA
tatgtggatggttttatttgcgcctagg

SEQ ID NO: 26933 - DNA, 28 bp, synthetic construct
  source 1..28: mol_type = other DNA
tcaaatagggtgaaaactatgtggatgg

SEQ ID NO: 26934 - DNA, 28 bp, synthetic construct
  source 1..28: mol_type = other DNA
gtgttcaaatagggtgaaaactatgtgg

SEQ ID NO: 26935 - DNA, 28 bp, synthetic construct
  source 1..28: mol_type = other DNA
catagttttcaccctatttgaacactgg

SEQ ID NO: 26936 - DNA, 28 bp, synthetic construct
  source 1..28: mol_type = other DNA
atttcaggtatgtaatttttatattagg

SEQ ID NO: 26937 - DNA, 28 bp, synthetic construct
  source 1..28: mol_type = other DNA
taaaaattacatacctgaaatcctatgg

SEQ ID NO: 26938 - DNA, 28 bp, synthetic construct
  source 1..28: mol_type = other DNA
tacatacctgaaatcctatggcacctgg

SEQ ID NO: 26939 - DNA, 28 bp, synthetic construct
  source 1..28: mol_type = other DNA
atgggaccaggtgccataggatttcagg

SEQ ID NO: 26940 - DNA, 28 bp, synthetic construct
  source 1..28: mol_type = other DNA
taaattttatgggaccaggtgccatagg

SEQ ID NO: 26941 - DNA, 28 bp, synthetic construct
  source 1..28: mol_type = other DNA
ttttaaaaataaattttatgggaccagg

SEQ ID NO: 26942 - DNA, 28 bp, synthetic construct
  source 1..28: mol_type = other DNA
tttttattttaaaaataaattttatggg

SEQ ID NO: 26943 - DNA, 28 bp, synthetic construct
  source 1..28: mol_type = other DNA
ttttttattttaaaaataaattttatgg

SEQ ID NO: 26944 - DNA, 28 bp, synthetic construct
  source 1..28: mol_type = other DNA
ttctataactacaggctgaaagatgagg

SEQ ID NO: 26945 - DNA, 28 bp, synthetic construct
  source 1..28: mol_type = other DNA
tttaattcataaatttttttatttaagg

SEQ ID NO: 26946 - DNA, 28 bp, synthetic construct
  source 1..28: mol_type = other DNA
cattgggttttcttaacttgaatatagg

SEQ ID NO: 26947 - DNA, 28 bp, synthetic construct
  source 1..28: mol_type = other DNA
ttcaaagagtgtatttgaatttttgtgg

SEQ ID NO: 26948 - DNA, 28 bp, synthetic construct
  source 1..28: mol_type = other DNA
aaatacactctttgaaacaaagacaagg

SEQ ID NO: 26949 - DNA, 28 bp, synthetic construct
  source 1..28: mol_type = other DNA
aatacactctttgaaacaaagacaaggg

SEQ ID NO: 26950 - DNA, 28 bp, synthetic construct
  source 1..28: mol_type = other DNA
tttgaaacaaagacaagggctcaagtgg

SEQ ID NO: 26951 - DNA, 28 bp, synthetic construct
  source 1..28: mol_type = other DNA
caaaaaatgagacaagtcttgttattgg

SEQ ID NO: 26952 - DNA, 28 bp, synthetic construct
  source 1..28: mol_type = other DNA
gagacaagtcttgttattggaacccagg

SEQ ID NO: 26953 - DNA, 28 bp, synthetic construct
  source 1..28: mol_type = other DNA
tgatcttgcattgattctgtttcctggg

SEQ ID NO: 26954 - DNA, 28 bp, synthetic construct
  source 1..28: mol_type = other DNA
atgatcttgcattgattctgtttcctgg

SEQ ID NO: 26955 - DNA, 28 bp, synthetic construct
  source 1..28: mol_type = other DNA
ggttaaattatcgttgttctttcagagg

SEQ ID NO: 26956 - DNA, 28 bp, synthetic construct
  source 1..28: mol_type = other DNA
agtttaagttgaaaaacctcagttctgg

SEQ ID NO: 26957 - DNA, 28 bp, synthetic construct
  source 1..28: mol_type = other DNA
gtttaagttgaaaaacctcagttctggg

SEQ ID NO: 26958 - DNA, 28 bp, synthetic construct
  source 1..28: mol_type = other DNA
actctgatgctgtatcccagaactgagg

SEQ ID NO: 26959 - DNA, 28 bp, synthetic construct
  source 1..28: mol_type = other DNA
agcatcagagtttattcactgccagtgg

SEQ ID NO: 26960 - DNA, 28 bp, synthetic construct
  source 1..28: mol_type = other DNA
atttttttttttaaattgcttccactgg

SEQ ID NO: 26961 - DNA, 28 bp, synthetic construct
  source 1..28: mol_type = other DNA
tcaccactctaaaaagtgaaaatcaagg

SEQ ID NO: 26962 - DNA, 28 bp, synthetic construct
  source 1..28: mol_type = other DNA
caccactctaaaaagtgaaaatcaaggg

SEQ ID NO: 26963 - DNA, 28 bp, synthetic construct
  source 1..28: mol_type = other DNA
ctcccttgattttcactttttagagtgg

SEQ ID NO: 26964 - DNA, 28 bp, synthetic construct
  source 1..28: mol_type = other DNA
tttatataattctttaaagccatatagg

SEQ ID NO: 26965 - DNA, 28 bp, synthetic construct
  source 1..28: mol_type = other DNA
aaaatcatagtataaacagcctatatgg

SEQ ID NO: 26966 - DNA, 28 bp, synthetic construct
  source 1..28: mol_type = other DNA
tggatttttttttttttttttgagatgg

SEQ ID NO: 26967 - DNA, 28 bp, synthetic construct
  source 1..28: mol_type = other DNA
agaagtcttaatttctactgcaaaatgg

SEQ ID NO: 26968 - DNA, 28 bp, synthetic construct
  source 1..28: mol_type = other DNA
ttctatgtcccagactcagtatataagg

SEQ ID NO: 26969 - DNA, 28 bp, synthetic construct
  source 1..28: mol_type = other DNA
gtattataccttatatactgagtctggg

SEQ ID NO: 26970 - DNA, 28 bp, synthetic construct
  source 1..28: mol_type = other DNA
agtattataccttatatactgagtctgg

SEQ ID NO: 26971 - DNA, 28 bp, synthetic construct
  source 1..28: mol_type = other DNA
tctccattacaaattaaaatgatcatgg

SEQ ID NO: 26972 - DNA, 28 bp, synthetic construct
  source 1..28: mol_type = other DNA
aaaccatgatcattttaatttgtaatgg

SEQ ID NO: 26973 - DNA, 28 bp, synthetic construct
  source 1..28: mol_type = other DNA
aagacatttatttttaaattaattatgg

SEQ ID NO: 26974 - DNA, 28 bp, synthetic construct
  source 1..28: mol_type = other DNA
tggtaagtgaacaaagccagactaaagg

SEQ ID NO: 26975 - DNA, 28 bp, synthetic construct
  source 1..28: mol_type = other DNA
ttgaagtttgataagcacatgcatttgg

SEQ ID NO: 26976 - DNA, 28 bp, synthetic construct
  source 1..28: mol_type = other DNA
aaccatcatataaagtccacaatttcgg

SEQ ID NO: 26977 - DNA, 28 bp, synthetic construct
  source 1..28: mol_type = other DNA
accatcatataaagtccacaatttcggg

SEQ ID NO: 26978 - DNA, 28 bp, synthetic construct
  source 1..28: mol_type = other DNA
gcccgaaattgtggactttatatgatgg

SEQ ID NO: 26979 - DNA, 28 bp, synthetic construct
  source 1..28: mol_type = other DNA
taaagtccacaatttcgggcaagaaagg

SEQ ID NO: 26980 - DNA, 28 bp, synthetic construct
  source 1..28: mol_type = other DNA
gtaagacctttcttgcccgaaattgtgg

SEQ ID NO: 26981 - DNA, 28 bp, synthetic construct
  source 1..28: mol_type = other DNA
ggtttgttttcattttttaactttatgg

SEQ ID NO: 26982 - DNA, 28 bp, synthetic construct
  source 1..28: mol_type = other DNA
tgaaaaaatatagcatgtatatatctgg

SEQ ID NO: 26983 - DNA, 28 bp, synthetic construct
  source 1..28: mol_type = other DNA
ttgaccgctagcctttagcaattaaagg

SEQ ID NO: 26984 - DNA, 28 bp, synthetic construct
  source 1..28: mol_type = other DNA
ttggcctttaattgctaaaggctagcgg

SEQ ID NO: 26985 - DNA, 28 bp, synthetic construct
  source 1..28: mol_type = other DNA
cttagttttggcctttaattgctaaagg

SEQ ID NO: 26986 - DNA, 28 bp, synthetic construct
  source 1..28: mol_type = other DNA
ctttagcaattaaaggccaaaactaagg

SEQ ID NO: 26987 - DNA, 28 bp, synthetic construct
  source 1..28: mol_type = other DNA
aaggccaaaactaaggaatgaatattgg

SEQ ID NO: 26988 - DNA, 28 bp, synthetic construct
  source 1..28: mol_type = other DNA
ggggccaatattcattccttagttttgg

SEQ ID NO: 26989 - DNA, 28 bp, synthetic construct
  source 1..28: mol_type = other DNA
ttagcatataaagattttcattttgggg

SEQ ID NO: 26990 - DNA, 28 bp, synthetic construct
  source 1..28: mol_type = other DNA
attagcatataaagattttcattttggg

SEQ ID NO: 26991 - DNA, 28 bp, synthetic construct
  source 1..28: mol_type = other DNA
cattagcatataaagattttcattttgg

SEQ ID NO: 26992 - DNA, 28 bp, synthetic construct
  source 1..28: mol_type = other DNA
ctgctctctctcctctctcttcacaggg

SEQ ID NO: 26993 - DNA, 28 bp, synthetic construct
  source 1..28: mol_type = other DNA
tctgctctctctcctctctcttcacagg

SEQ ID NO: 26994 - DNA, 28 bp, synthetic construct
  source 1..28: mol_type = other DNA
gaagagagaggagagagagcagatgagg

SEQ ID NO: 26995 - DNA, 28 bp, synthetic construct
  source 1..28: mol_type = other DNA
aagagagaggagagagagcagatgaggg

SEQ ID NO: 26996 - DNA, 28 bp, synthetic construct
  source 1..28: mol_type = other DNA
atgagggaagcagacagaaagagcaagg

SEQ ID NO: 26997 - DNA, 28 bp, synthetic construct
  source 1..28: mol_type = other DNA
aagcagacagaaagagcaaggctccagg

SEQ ID NO: 26998 - DNA, 28 bp, synthetic construct
  source 1..28: mol_type = other DNA
agacagaaagagcaaggctccaggaagg

SEQ ID NO: 26999 - DNA, 28 bp, synthetic construct
  source 1..28: mol_type = other DNA
aggagcagacttaacaaggccttcctgg

SEQ ID NO: 27000 - DNA, 28 bp, synthetic construct
  source 1..28: mol_type = other DNA
aggaaggccttgttaagtctgctcctgg

SEQ ID NO: 27001 - DNA, 28 bp, synthetic construct
  source 1..28: mol_type = other DNA
ggaaggccttgttaagtctgctcctggg

SEQ ID NO: 27002 - DNA, 28 bp, synthetic construct
  source 1..28: mol_type = other DNA
taacatcccaggagcagacttaacaagg

SEQ ID NO: 27003 - DNA, 28 bp, synthetic construct
  source 1..28: mol_type = other DNA
tcctgggatgttacaagacagacagcgg

SEQ ID NO: 27004 - DNA, 28 bp, synthetic construct
  source 1..28: mol_type = other DNA
tccgctgtctgtcttgtaacatcccagg

SEQ ID NO: 27005 - DNA, 28 bp, synthetic construct
  source 1..28: mol_type = other DNA
gggatgttacaagacagacagcggacgg

SEQ ID NO: 27006 - DNA, 28 bp, synthetic construct
  source 1..28: mol_type = other DNA
ggatgttacaagacagacagcggacggg

SEQ ID NO: 27007 - DNA, 28 bp, synthetic construct
  source 1..28: mol_type = other DNA
atcttgacttcttttggaaatgaaatgg

SEQ ID NO: 27008 - DNA, 28 bp, synthetic construct
  source 1..28: mol_type = other DNA
ggtaaaagtatatcttgacttcttttgg

SEQ ID NO: 27009 - DNA, 28 bp, synthetic construct
  source 1..28: mol_type = other DNA
ttgtgcttgttctgctttaaatcatagg

SEQ ID NO: 27010 - DNA, 28 bp, synthetic construct
  source 1..28: mol_type = other DNA
aacacatcattttcagacatttgcgtgg

SEQ ID NO: 27011 - DNA, 28 bp, synthetic construct
  source 1..28: mol_type = other DNA
aacagtaattttgaaatgacagttgtgg

SEQ ID NO: 27012 - DNA, 28 bp, synthetic construct
  source 1..28: mol_type = other DNA
gtttttatcttcatattaatattctagg

SEQ ID NO: 27013 - DNA, 28 bp, synthetic construct
  source 1..28: mol_type = other DNA
gatccatattcatatgcacttcataggg

SEQ ID NO: 27014 - DNA, 28 bp, synthetic construct
  source 1..28: mol_type = other DNA
tgatccatattcatatgcacttcatagg

SEQ ID NO: 27015 - DNA, 28 bp, synthetic construct
  source 1..28: mol_type = other DNA
gatcacacccatcgcactgtcactcagg

SEQ ID NO: 27016 - DNA, 28 bp, synthetic construct
  source 1..28: mol_type = other DNA
atcacacccatcgcactgtcactcaggg

SEQ ID NO: 27017 - DNA, 28 bp, synthetic construct
  source 1..28: mol_type = other DNA
tgacttccctgagtgacagtgcgatggg

SEQ ID NO: 27018 - DNA, 28 bp, synthetic construct
  source 1..28: mol_type = other DNA
ttgacttccctgagtgacagtgcgatgg

SEQ ID NO: 27019 - DNA, 28 bp, synthetic construct
  source 1..28: mol_type = other DNA
gtaatctcttaaattgcacaaatctagg

SEQ ID NO: 27020 - DNA, 28 bp, synthetic construct
  source 1..28: mol_type = other DNA
caccttttcacgttgctctccactcagg

SEQ ID NO: 27021 - DNA, 28 bp, synthetic construct
  source 1..28: mol_type = other DNA
cacctgagtggagagcaacgtgaaaagg

SEQ ID NO: 27022 - DNA, 28 bp, synthetic construct
  source 1..28: mol_type = other DNA
agaggagttggaagtcacacctgagtgg

SEQ ID NO: 27023 - DNA, 28 bp, synthetic construct
  source 1..28: mol_type = other DNA
agtggggtttatgtgagagaggagttgg

SEQ ID NO: 27024 - DNA, 28 bp, synthetic construct
  source 1..28: mol_type = other DNA
cacagaagtggggtttatgtgagagagg

SEQ ID NO: 27025 - DNA, 28 bp, synthetic construct
  source 1..28: mol_type = other DNA
catggactgcatcggcacagaagtgggg

SEQ ID NO: 27026 - DNA, 28 bp, synthetic construct
  source 1..28: mol_type = other DNA
tcatggactgcatcggcacagaagtggg

SEQ ID NO: 27027 - DNA, 28 bp, synthetic construct
  source 1..28: mol_type = other DNA
gtcatggactgcatcggcacagaagtgg

SEQ ID NO: 27028 - DNA, 28 bp, synthetic construct
  source 1..28: mol_type = other DNA
agagaagatatgtcatggactgcatcgg

SEQ ID NO: 27029 - DNA, 28 bp, synthetic construct
  source 1..28: mol_type = other DNA
gcgtctagttagagaagatatgtcatgg

SEQ ID NO: 27030 - DNA, 28 bp, synthetic construct
  source 1..28: mol_type = other DNA
tatcttctctaactagacgctctgatgg

SEQ ID NO: 27031 - DNA, 28 bp, synthetic construct
  source 1..28: mol_type = other DNA
ctgatggaatgcctccatgatgaactgg

SEQ ID NO: 27032 - DNA, 28 bp, synthetic construct
  source 1..28: mol_type = other DNA
cagggaacagaccagttcatcatggagg

SEQ ID NO: 27033 - DNA, 28 bp, synthetic construct
  source 1..28: mol_type = other DNA
atgcagggaacagaccagttcatcatgg

SEQ ID NO: 27034 - DNA, 28 bp, synthetic construct
  source 1..28: mol_type = other DNA
atgattgctgaaagtattcaatgcaggg

SEQ ID NO: 27035 - DNA, 28 bp, synthetic construct
  source 1..28: mol_type = other DNA
tatgattgctgaaagtattcaatgcagg

SEQ ID NO: 27036 - DNA, 28 bp, synthetic construct
  source 1..28: mol_type = other DNA
agtcaacaaacatattttaacctatagg

SEQ ID NO: 27037 - DNA, 28 bp, synthetic construct
  source 1..28: mol_type = other DNA
gtcaacaaacatattttaacctataggg

SEQ ID NO: 27038 - DNA, 28 bp, synthetic construct
  source 1..28: mol_type = other DNA
catattttaacctatagggatctaaagg

SEQ ID NO: 27039 - DNA, 28 bp, synthetic construct
  source 1..28: mol_type = other DNA
taatgtcttacctttagatccctatagg

SEQ ID NO: 27040 - DNA, 28 bp, synthetic construct
  source 1..28: mol_type = other DNA
cattatttgtttgaagcttttaaaaagg

SEQ ID NO: 27041 - DNA, 28 bp, synthetic construct
  source 1..28: mol_type = other DNA
aataaagtatcagtactcagagtcacgg

SEQ ID NO: 27042 - DNA, 28 bp, synthetic construct
  source 1..28: mol_type = other DNA
tgatactttattgcataaaatattgtgg

SEQ ID NO: 27043 - DNA, 28 bp, synthetic construct
  source 1..28: mol_type = other DNA
gatactttattgcataaaatattgtggg

SEQ ID NO: 27044 - DNA, 28 bp, synthetic construct
  source 1..28: mol_type = other DNA
ctttattgcataaaatattgtgggaagg

SEQ ID NO: 27045 - DNA, 28 bp, synthetic construct
  source 1..28: mol_type = other DNA
gagcttgagtagttgctacctgaatagg

SEQ ID NO: 27046 - DNA, 28 bp, synthetic construct
  source 1..28: mol_type = other DNA
cctgaataggcctagtgagatcagcagg

SEQ ID NO: 27047 - DNA, 28 bp, synthetic construct
  source 1..28: mol_type = other DNA
aataggcctagtgagatcagcaggaagg

SEQ ID NO: 27048 - DNA, 28 bp, synthetic construct
  source 1..28: mol_type = other DNA
ataggcctagtgagatcagcaggaaggg

SEQ ID NO: 27049 - DNA, 28 bp, synthetic construct
  source 1..28: mol_type = other DNA
taggcctagtgagatcagcaggaagggg

SEQ ID NO: 27050 - DNA, 28 bp, synthetic construct
  source 1..28: mol_type = other DNA
atttccccttcctgctgatctcactagg

SEQ ID NO: 27051 - DNA, 28 bp, synthetic construct
  source 1..28: mol_type = other DNA
cagcaggaaggggaaattccagcagagg

SEQ ID NO: 27052 - DNA, 28 bp, synthetic construct
  source 1..28: mol_type = other DNA
agcaggaaggggaaattccagcagaggg

SEQ ID NO: 27053 - DNA, 28 bp, synthetic construct
  source 1..28: mol_type = other DNA
ttccagcagagggcacatcataaagagg

SEQ ID NO: 27054 - DNA, 28 bp, synthetic construct
  source 1..28: mol_type = other DNA
ttcctctttatgatgtgccctctgctgg

SEQ ID NO: 27055 - DNA, 28 bp, synthetic construct
  source 1..28: mol_type = other DNA
agggcacatcataaagaggaatgaaagg

SEQ ID NO: 27056 - DNA, 28 bp, synthetic construct
  source 1..28: mol_type = other DNA
gggcacatcataaagaggaatgaaaggg

SEQ ID NO: 27057 - DNA, 28 bp, synthetic construct
  source 1..28: mol_type = other DNA
catcataaagaggaatgaaagggaatgg

SEQ ID NO: 27058 - DNA, 28 bp, synthetic construct
  source 1..28: mol_type = other DNA
agaggaatgaaagggaatggtgtagcgg

SEQ ID NO: 27059 - DNA, 28 bp, synthetic construct
  source 1..28: mol_type = other DNA
gaatgaaagggaatggtgtagcggcagg

SEQ ID NO: 27060 - DNA, 28 bp, synthetic construct
  source 1..28: mol_type = other DNA
aaagggaatggtgtagcggcaggactgg

SEQ ID NO: 27061 - DNA, 28 bp, synthetic construct
  source 1..28: mol_type = other DNA
agcggcaggactggcagattcagaaagg

SEQ ID NO: 27062 - DNA, 28 bp, synthetic construct
  source 1..28: mol_type = other DNA
gcaggactggcagattcagaaaggctgg

SEQ ID NO: 27063 - DNA, 28 bp, synthetic construct
  source 1..28: mol_type = other DNA
ggcagattcagaaaggctggcgagctgg

SEQ ID NO: 27064 - DNA, 28 bp, synthetic construct
  source 1..28: mol_type = other DNA
agaaaggctggcgagctggctagagagg

SEQ ID NO: 27065 - DNA, 28 bp, synthetic construct
  source 1..28: mol_type = other DNA
gaaaggctggcgagctggctagagaggg

SEQ ID NO: 27066 - DNA, 28 bp, synthetic construct
  source 1..28: mol_type = other DNA
tagagagggctccccagacacattaagg

SEQ ID NO: 27067 - DNA, 28 bp, synthetic construct
  source 1..28: mol_type = other DNA
agagagggctccccagacacattaaggg

SEQ ID NO: 27068 - DNA, 28 bp, synthetic construct
  source 1..28: mol_type = other DNA
gagggctccccagacacattaagggcgg

SEQ ID NO: 27069 - DNA, 28 bp, synthetic construct
  source 1..28: mol_type = other DNA
tcagggtccgcccttaatgtgtctgggg

SEQ ID NO: 27070 - DNA, 28 bp, synthetic construct
  source 1..28: mol_type = other DNA
ttcagggtccgcccttaatgtgtctggg

SEQ ID NO: 27071 - DNA, 28 bp, synthetic construct
  source 1..28: mol_type = other DNA
cttcagggtccgcccttaatgtgtctgg

SEQ ID NO: 27072 - DNA, 28 bp, synthetic construct
  source 1..28: mol_type = other DNA
cagacacattaagggcggaccctgaagg

SEQ ID NO: 27073 - DNA, 28 bp, synthetic construct
  source 1..28: mol_type = other DNA
agacacattaagggcggaccctgaaggg

SEQ ID NO: 27074 - DNA, 28 bp, synthetic construct
  source 1..28: mol_type = other DNA
ttaagggcggaccctgaagggcacgtgg

SEQ ID NO: 27075 - DNA, 28 bp, synthetic construct
  source 1..28: mol_type = other DNA
taagggcggaccctgaagggcacgtggg

SEQ ID NO: 27076 - DNA, 28 bp, synthetic construct
  source 1..28: mol_type = other DNA
tgtagcacggcccacgtgcccttcaggg

SEQ ID NO: 27077 - DNA, 28 bp, synthetic construct
  source 1..28: mol_type = other DNA
ctgtagcacggcccacgtgcccttcagg

SEQ ID NO: 27078 - DNA, 28 bp, synthetic construct
  source 1..28: mol_type = other DNA
ctgaagggcacgtgggccgtgctacagg

SEQ ID NO: 27079 - DNA, 28 bp, synthetic construct
  source 1..28: mol_type = other DNA
ggcacgtgggccgtgctacaggcacagg

SEQ ID NO: 27080 - DNA, 28 bp, synthetic construct
  source 1..28: mol_type = other DNA
tgggccgtgctacaggcacaggctctgg

SEQ ID NO: 27081 - DNA, 28 bp, synthetic construct
  source 1..28: mol_type = other DNA
ctgtccagagcctgtgcctgtagcacgg

SEQ ID NO: 27082 - DNA, 28 bp, synthetic construct
  source 1..28: mol_type = other DNA
cgtgctacaggcacaggctctggacagg

SEQ ID NO: 27083 - DNA, 28 bp, synthetic construct
  source 1..28: mol_type = other DNA
gtgctacaggcacaggctctggacaggg

SEQ ID NO: 27084 - DNA, 28 bp, synthetic construct
  source 1..28: mol_type = other DNA
acagggccccagtgaagttctttaaagg

SEQ ID NO: 27085 - DNA, 28 bp, synthetic construct
  source 1..28: mol_type = other DNA
gccccagtgaagttctttaaaggactgg

SEQ ID NO: 27086 - DNA, 28 bp, synthetic construct
  source 1..28: mol_type = other DNA
accagtcctttaaagaacttcactgggg

SEQ ID NO: 27087 - DNA, 28 bp, synthetic construct
  source 1..28: mol_type = other DNA
taccagtcctttaaagaacttcactggg

SEQ ID NO: 27088 - DNA, 28 bp, synthetic construct
  source 1..28: mol_type = other DNA
ataccagtcctttaaagaacttcactgg

SEQ ID NO: 27089 - DNA, 28 bp, synthetic construct
  source 1..28: mol_type = other DNA
aaataactctcagcagcatagaagatgg

SEQ ID NO: 27090 - DNA, 28 bp, synthetic construct
  source 1..28: mol_type = other DNA
tagaagatggactgaaccaagaagaagg

SEQ ID NO: 27091 - DNA, 28 bp, synthetic construct
  source 1..28: mol_type = other DNA
ttggtgtatgaagttgccttcttcttgg

SEQ ID NO: 27092 - DNA, 28 bp, synthetic construct
  source 1..28: mol_type = other DNA
ccttttgattacgctttcagtgtattgg

SEQ ID NO: 27093 - DNA, 28 bp, synthetic construct
  source 1..28: mol_type = other DNA
ctgaaagcgtaatcaaaaggtgatgagg

SEQ ID NO: 27094 - DNA, 28 bp, synthetic construct
  source 1..28: mol_type = other DNA
aggtgatgaggcctgaatcaagtagtgg

SEQ ID NO: 27095 - DNA, 28 bp, synthetic construct
  source 1..28: mol_type = other DNA
tgatgaggcctgaatcaagtagtggcgg

SEQ ID NO: 27096 - DNA, 28 bp, synthetic construct
  source 1..28: mol_type = other DNA
tgaggcctgaatcaagtagtggcggtgg

SEQ ID NO: 27097 - DNA, 28 bp, synthetic construct
  source 1..28: mol_type = other DNA
gaggcctgaatcaagtagtggcggtggg

SEQ ID NO: 27098 - DNA, 28 bp, synthetic construct
  source 1..28: mol_type = other DNA
cattcccaccgccactacttgattcagg

SEQ ID NO: 27099 - DNA, 28 bp, synthetic construct
  source 1..28: mol_type = other DNA
ggtgggaatgtaaagagtatttccaagg

SEQ ID NO: 27100 - DNA, 28 bp, synthetic construct
  source 1..28: mol_type = other DNA
tagcaaagctgtgatggtgctaccttgg

SEQ ID NO: 27101 - DNA, 28 bp, synthetic construct
  source 1..28: mol_type = other DNA
gtatactttattagcaaagctgtgatgg

SEQ ID NO: 27102 - DNA, 28 bp, synthetic construct
  source 1..28: mol_type = other DNA
tttgctaataaagtatacattgtttagg

SEQ ID NO: 27103 - DNA, 28 bp, synthetic construct
  source 1..28: mol_type = other DNA
aagtatacattgtttaggaaacatttgg

SEQ ID NO: 27104 - DNA, 28 bp, synthetic construct
  source 1..28: mol_type = other DNA
aggacagtaaactattgtttggaaaagg

SEQ ID NO: 27105 - DNA, 28 bp, synthetic construct
  source 1..28: mol_type = other DNA
atttcaaggacagtaaactattgtttgg

SEQ ID NO: 27106 - DNA, 28 bp, synthetic construct
  source 1..28: mol_type = other DNA
gggttgaaagacgctgatgatttcaagg

SEQ ID NO: 27107 - DNA, 28 bp, synthetic construct
  source 1..28: mol_type = other DNA
aagtttaggatcttgaaatcatgatggg

SEQ ID NO: 27108 - DNA, 28 bp, synthetic construct
  source 1..28: mol_type = other DNA
caagtttaggatcttgaaatcatgatgg

SEQ ID NO: 27109 - DNA, 28 bp, synthetic construct
  source 1..28: mol_type = other DNA
atgatttcaagatcctaaacttgacagg

SEQ ID NO: 27110 - DNA, 28 bp, synthetic construct
  source 1..28: mol_type = other DNA
ttagtgacattgtcctgtcaagtttagg

SEQ ID NO: 27111 - DNA, 28 bp, synthetic construct
  source 1..28: mol_type = other DNA
aggactttttcaattaggagatttgtgg

SEQ ID NO: 27112 - DNA, 28 bp, synthetic construct
  source 1..28: mol_type = other DNA
cagattaaagaggactttttcaattagg

SEQ ID NO: 27113 - DNA, 28 bp, synthetic construct
  source 1..28: mol_type = other DNA
gcagactcttggggacagattaaagagg

SEQ ID NO: 27114 - DNA, 28 bp, synthetic construct
  source 1..28: mol_type = other DNA
gtattcttttcattgcagactcttgggg

SEQ ID NO: 27115 - DNA, 28 bp, synthetic construct
  source 1..28: mol_type = other DNA
ggtattcttttcattgcagactcttggg

SEQ ID NO: 27116 - DNA, 28 bp, synthetic construct
  source 1..28: mol_type = other DNA
aggtattcttttcattgcagactcttgg

SEQ ID NO: 27117 - DNA, 28 bp, synthetic construct
  source 1..28: mol_type = other DNA
tacctgagaaatgtctttacaaaatagg

SEQ ID NO: 27118 - DNA, 28 bp, synthetic construct
  source 1..28: mol_type = other DNA
tacctattttgtaaagacatttctcagg

SEQ ID NO: 27119 - DNA, 28 bp, synthetic construct
  source 1..28: mol_type = other DNA
acaaaataggtaaaattcattagtttgg

SEQ ID NO: 27120 - DNA, 28 bp, synthetic construct
  source 1..28: mol_type = other DNA
ttggaaaacagacatttttcctctttgg

SEQ ID NO: 27121 - DNA, 28 bp, synthetic construct
  source 1..28: mol_type = other DNA
tcttattttatacaagctaccaaagagg

SEQ ID NO: 27122 - DNA, 28 bp, synthetic construct
  source 1..28: mol_type = other DNA
tcaccatttttttttttttttgagatgg

SEQ ID NO: 27123 - DNA, 28 bp, synthetic construct
  source 1..28: mol_type = other DNA
actccatctcaaaaaaaaaaaaaaatgg

SEQ ID NO: 27124 - DNA, 28 bp, synthetic construct
  source 1..28: mol_type = other DNA
agatggagtttcgctcttgttgcccagg

SEQ ID NO: 27125 - DNA, 28 bp, synthetic construct
  source 1..28: mol_type = other DNA
ggagtttcgctcttgttgcccaggctgg

SEQ ID NO: 27126 - DNA, 28 bp, synthetic construct
  source 1..28: mol_type = other DNA
tcttgttgcccaggctggagtgcaatgg

SEQ ID NO: 27127 - DNA, 28 bp, synthetic construct
  source 1..28: mol_type = other DNA
agatcgcaccattgcactccagcctggg

SEQ ID NO: 27128 - DNA, 28 bp, synthetic construct
  source 1..28: mol_type = other DNA
gagatcgcaccattgcactccagcctgg

SEQ ID NO: 27129 - DNA, 28 bp, synthetic construct
  source 1..28: mol_type = other DNA
tcagttcaccacaacctccacctcctgg

SEQ ID NO: 27130 - DNA, 28 bp, synthetic construct
  source 1..28: mol_type = other DNA
cagttcaccacaacctccacctcctggg

SEQ ID NO: 27131 - DNA, 28 bp, synthetic construct
  source 1..28: mol_type = other DNA
gcttgaacccaggaggtggaggttgtgg

SEQ ID NO: 27132 - DNA, 28 bp, synthetic construct
  source 1..28: mol_type = other DNA
agaattgcttgaacccaggaggtggagg

SEQ ID NO: 27133 - DNA, 28 bp, synthetic construct
  source 1..28: mol_type = other DNA
aggagaattgcttgaacccaggaggtgg

SEQ ID NO: 27134 - DNA, 28 bp, synthetic construct
  source 1..28: mol_type = other DNA
ggcaggagaattgcttgaacccaggagg

SEQ ID NO: 27135 - DNA, 28 bp, synthetic construct
  source 1..28: mol_type = other DNA
tgaggcaggagaattgcttgaacccagg

SEQ ID NO: 27136 - DNA, 28 bp, synthetic construct
  source 1..28: mol_type = other DNA
ctcctgcctcagcctcctgagtagctgg

SEQ ID NO: 27137 - DNA, 28 bp, synthetic construct
  source 1..28: mol_type = other DNA
tcctgcctcagcctcctgagtagctggg

SEQ ID NO: 27138 - DNA, 28 bp, synthetic construct
  source 1..28: mol_type = other DNA
tcccagctactcaggaggctgaggcagg

SEQ ID NO: 27139 - DNA, 28 bp, synthetic construct
  source 1..28: mol_type = other DNA
gtaatcccagctactcaggaggctgagg

SEQ ID NO: 27140 - DNA, 28 bp, synthetic construct
  source 1..28: mol_type = other DNA
cagcctcctgagtagctgggattacagg

SEQ ID NO: 27141 - DNA, 28 bp, synthetic construct
  source 1..28: mol_type = other DNA
atgcctgtaatcccagctactcaggagg

SEQ ID NO: 27142 - DNA, 28 bp, synthetic construct
  source 1..28: mol_type = other DNA
cacatgcctgtaatcccagctactcagg

SEQ ID NO: 27143 - DNA, 28 bp, synthetic construct
  source 1..28: mol_type = other DNA
aaaatacaaaattagctgggcgtggtgg

SEQ ID NO: 27144 - DNA, 28 bp, synthetic construct
  source 1..28: mol_type = other DNA
ctaaaaatacaaaattagctgggcgtgg

SEQ ID NO: 27145 - DNA, 28 bp, synthetic construct
  source 1..28: mol_type = other DNA
ctctgctaaaaatacaaaattagctggg

SEQ ID NO: 27146 - DNA, 28 bp, synthetic construct
  source 1..28: mol_type = other DNA
tctctgctaaaaatacaaaattagctgg

SEQ ID NO: 27147 - DNA, 28 bp, synthetic construct
  source 1..28: mol_type = other DNA
gctaattttgtatttttagcagagacgg

SEQ ID NO: 27148 - DNA, 28 bp, synthetic construct
  source 1..28: mol_type = other DNA
ctaattttgtatttttagcagagacggg

SEQ ID NO: 27149 - DNA, 28 bp, synthetic construct
  source 1..28: mol_type = other DNA
taattttgtatttttagcagagacgggg

SEQ ID NO: 27150 - DNA, 28 bp, synthetic construct
  source 1..28: mol_type = other DNA
tagcagagacggggtttctccatgttgg

SEQ ID NO: 27151 - DNA, 28 bp, synthetic construct
  source 1..28: mol_type = other DNA
gagacggggtttctccatgttggtcagg

SEQ ID NO: 27152 - DNA, 28 bp, synthetic construct
  source 1..28: mol_type = other DNA
cggggtttctccatgttggtcaggctgg

SEQ ID NO: 27153 - DNA, 28 bp, synthetic construct
  source 1..28: mol_type = other DNA
gagttcaagaccagcctgaccaacatgg

SEQ ID NO: 27154 - DNA, 28 bp, synthetic construct
  source 1..28: mol_type = other DNA
aggctggtcttgaactctcgacctcagg

SEQ ID NO: 27155 - DNA, 28 bp, synthetic construct
  source 1..28: mol_type = other DNA
tcgacctcaggtgatccacctgcctcgg

SEQ ID NO: 27156 - DNA, 28 bp, synthetic construct
  source 1..28: mol_type = other DNA
gaggccgaggcaggtggatcacctgagg

SEQ ID NO: 27157 - DNA, 28 bp, synthetic construct
  source 1..28: mol_type = other DNA
caacactttgggaggccgaggcaggtgg

SEQ ID NO: 27158 - DNA, 28 bp, synthetic construct
  source 1..28: mol_type = other DNA
cacctgcctcggcctcccaaagtgttgg

SEQ ID NO: 27159 - DNA, 28 bp, synthetic construct
  source 1..28: mol_type = other DNA
acctgcctcggcctcccaaagtgttggg

SEQ ID NO: 27160 - DNA, 28 bp, synthetic construct
  source 1..28: mol_type = other DNA
tcccaacactttgggaggccgaggcagg

SEQ ID NO: 27161 - DNA, 28 bp, synthetic construct
  source 1..28: mol_type = other DNA
gtaatcccaacactttgggaggccgagg

SEQ ID NO: 27162 - DNA, 28 bp, synthetic construct
  source 1..28: mol_type = other DNA
cggcctcccaaagtgttgggattacagg

SEQ ID NO: 27163 - DNA, 28 bp, synthetic construct
  source 1..28: mol_type = other DNA
actcctgtaatcccaacactttgggagg

SEQ ID NO: 27164 - DNA, 28 bp, synthetic construct
  source 1..28: mol_type = other DNA
ctcactcctgtaatcccaacactttggg

SEQ ID NO: 27165 - DNA, 28 bp, synthetic construct
  source 1..28: mol_type = other DNA
gctcactcctgtaatcccaacactttgg

SEQ ID NO: 27166 - DNA, 28 bp, synthetic construct
  source 1..28: mol_type = other DNA
gtgttgggattacaggagtgagccacgg

SEQ ID NO: 27167 - DNA, 28 bp, synthetic construct
  source 1..28: mol_type = other DNA
aatggtgcaatactgctgagcgccgtgg

SEQ ID NO: 27168 - DNA, 28 bp, synthetic construct
  source 1..28: mol_type = other DNA
cggagagtctgagtttcaaagaaaatgg

SEQ ID NO: 27169 - DNA, 28 bp, synthetic construct
  source 1..28: mol_type = other DNA
tttgaaactcagactctccgcttctagg

SEQ ID NO: 27170 - DNA, 28 bp, synthetic construct
  source 1..28: mol_type = other DNA
gtttaggctctaactctcctagaagcgg

SEQ ID NO: 27171 - DNA, 28 bp, synthetic construct
  source 1..28: mol_type = other DNA
gagagttagagcctaaacaaattgaagg

SEQ ID NO: 27172 - DNA, 28 bp, synthetic construct
  source 1..28: mol_type = other DNA
agttagagcctaaacaaattgaaggtgg

SEQ ID NO: 27173 - DNA, 28 bp, synthetic construct
  source 1..28: mol_type = other DNA
tagagcctaaacaaattgaaggtggagg

SEQ ID NO: 27174 - DNA, 28 bp, synthetic construct
  source 1..28: mol_type = other DNA
agagcctaaacaaattgaaggtggaggg

SEQ ID NO: 27175 - DNA, 28 bp, synthetic construct
  source 1..28: mol_type = other DNA
aagtccctccaccttcaatttgtttagg

SEQ ID NO: 27176 - DNA, 28 bp, synthetic construct
  source 1..28: mol_type = other DNA
aaacaaattgaaggtggagggacttagg

SEQ ID NO: 27177 - DNA, 28 bp, synthetic construct
  source 1..28: mol_type = other DNA
aacaaattgaaggtggagggacttaggg

SEQ ID NO: 27178 - DNA, 28 bp, synthetic construct
  source 1..28: mol_type = other DNA
acaaattgaaggtggagggacttagggg

SEQ ID NO: 27179 - DNA, 28 bp, synthetic construct
  source 1..28: mol_type = other DNA
aagatttaactttcatcacatccaaagg

SEQ ID NO: 27180 - DNA, 28 bp, synthetic construct
  source 1..28: mol_type = other DNA
gtttgcatggtgtctcatgggcctttgg

SEQ ID NO: 27181 - DNA, 28 bp, synthetic construct
  source 1..28: mol_type = other DNA
cccatgagacaccatgcaaacaatgcgg

SEQ ID NO: 27182 - DNA, 28 bp, synthetic construct
  source 1..28: mol_type = other DNA
tccgcattgtttgcatggtgtctcatgg

SEQ ID NO: 27183 - DNA, 28 bp, synthetic construct
  source 1..28: mol_type = other DNA
agatatttggtccgcattgtttgcatgg

SEQ ID NO: 27184 - DNA, 28 bp, synthetic construct
  source 1..28: mol_type = other DNA
aacaatgcggaccaaatatctatattgg

SEQ ID NO: 27185 - DNA, 28 bp, synthetic construct
  source 1..28: mol_type = other DNA
ttgctatatcaccaatatagatatttgg

SEQ ID NO: 27186 - DNA, 28 bp, synthetic construct
  source 1..28: mol_type = other DNA
aataaatgctaagaaaaaagagtaacgg

SEQ ID NO: 27187 - DNA, 28 bp, synthetic construct
  source 1..28: mol_type = other DNA
ataaatgctaagaaaaaagagtaacggg

SEQ ID NO: 27188 - DNA, 28 bp, synthetic construct
  source 1..28: mol_type = other DNA
aaaagagtaacgggactcacagcgctgg

SEQ ID NO: 27189 - DNA, 28 bp, synthetic construct
  source 1..28: mol_type = other DNA
aaagagtaacgggactcacagcgctggg

SEQ ID NO: 27190 - DNA, 28 bp, synthetic construct
  source 1..28: mol_type = other DNA
aagagtaacgggactcacagcgctgggg

SEQ ID NO: 27191 - DNA, 28 bp, synthetic construct
  source 1..28: mol_type = other DNA
taacgggactcacagcgctggggagagg

SEQ ID NO: 27192 - DNA, 28 bp, synthetic construct
  source 1..28: mol_type = other DNA
aacgggactcacagcgctggggagaggg

SEQ ID NO: 27193 - DNA, 28 bp, synthetic construct
  source 1..28: mol_type = other DNA
acgggactcacagcgctggggagagggg

SEQ ID NO: 27194 - DNA, 28 bp, synthetic construct
  source 1..28: mol_type = other DNA
gactcacagcgctggggagaggggcagg

SEQ ID NO: 27195 - DNA, 28 bp, synthetic construct
  source 1..28: mol_type = other DNA
agaggggcaggttgcaattctaaacagg

SEQ ID NO: 27196 - DNA, 28 bp, synthetic construct
  source 1..28: mol_type = other DNA
gaggggcaggttgcaattctaaacaggg

SEQ ID NO: 27197 - DNA, 28 bp, synthetic construct
  source 1..28: mol_type = other DNA
gggcaggttgcaattctaaacagggtgg

SEQ ID NO: 27198 - DNA, 28 bp, synthetic construct
  source 1..28: mol_type = other DNA
ggttgcaattctaaacagggtggtcagg

SEQ ID NO: 27199 - DNA, 28 bp, synthetic construct
  source 1..28: mol_type = other DNA
aggatgtagtgaaaaggagggcttgggg

SEQ ID NO: 27200 - DNA, 28 bp, synthetic construct
  source 1..28: mol_type = other DNA
caggatgtagtgaaaaggagggcttggg

SEQ ID NO: 27201 - DNA, 28 bp, synthetic construct
  source 1..28: mol_type = other DNA
gcaggatgtagtgaaaaggagggcttgg

SEQ ID NO: 27202 - DNA, 28 bp, synthetic construct
  source 1..28: mol_type = other DNA
aggaggcaggatgtagtgaaaaggaggg

SEQ ID NO: 27203 - DNA, 28 bp, synthetic construct
  source 1..28: mol_type = other DNA
taggaggcaggatgtagtgaaaaggagg

SEQ ID NO: 27204 - DNA, 28 bp, synthetic construct
  source 1..28: mol_type = other DNA
ttttaggaggcaggatgtagtgaaaagg

SEQ ID NO: 27205 - DNA, 28 bp, synthetic construct
  source 1..28: mol_type = other DNA
tattttttggtttgttttaggaggcagg

SEQ ID NO: 27206 - DNA, 28 bp, synthetic construct
  source 1..28: mol_type = other DNA
tgtgtattttttggtttgttttaggagg

SEQ ID NO: 27207 - DNA, 28 bp, synthetic construct
  source 1..28: mol_type = other DNA
gcatgtgtattttttggtttgttttagg

SEQ ID NO: 27208 - DNA, 28 bp, synthetic construct
  source 1..28: mol_type = other DNA
tgggtttgtgtgcatgtgtattttttgg

SEQ ID NO: 27209 - DNA, 28 bp, synthetic construct
  source 1..28: mol_type = other DNA
gcacacaaacccacaagtacttacatgg

SEQ ID NO: 27210 - DNA, 28 bp, synthetic construct
  source 1..28: mol_type = other DNA
cacacaaacccacaagtacttacatggg

SEQ ID NO: 27211 - DNA, 28 bp, synthetic construct
  source 1..28: mol_type = other DNA
gatgtaagcccatgtaagtacttgtggg

SEQ ID NO: 27212 - DNA, 28 bp, synthetic construct
  source 1..28: mol_type = other DNA
agatgtaagcccatgtaagtacttgtgg

SEQ ID NO: 27213 - DNA, 28 bp, synthetic construct
  source 1..28: mol_type = other DNA
attaaaatatatttttgttattttaagg

SEQ ID NO: 27214 - DNA, 28 bp, synthetic construct
  source 1..28: mol_type = other DNA
aagttttgctgtggagaatttaagaggg

SEQ ID NO: 27215 - DNA, 28 bp, synthetic construct
  source 1..28: mol_type = other DNA
taagttttgctgtggagaatttaagagg

SEQ ID NO: 27216 - DNA, 28 bp, synthetic construct
  source 1..28: mol_type = other DNA
ctggctgggaagataagttttgctgtgg

SEQ ID NO: 27217 - DNA, 28 bp, synthetic construct
  source 1..28: mol_type = other DNA
tgcttcatgttattttacgctggctggg

SEQ ID NO: 27218 - DNA, 28 bp, synthetic construct
  source 1..28: mol_type = other DNA
gtgcttcatgttattttacgctggctgg

SEQ ID NO: 27219 - DNA, 28 bp, synthetic construct
  source 1..28: mol_type = other DNA
ataagtgcttcatgttattttacgctgg

SEQ ID NO: 27220 - DNA, 28 bp, synthetic construct
  source 1..28: mol_type = other DNA
agcacttatgatatgccaagtactatgg

SEQ ID NO: 27221 - DNA, 28 bp, synthetic construct
  source 1..28: mol_type = other DNA
taaacaatgtgctttccatagtacttgg

SEQ ID NO: 27222 - DNA, 28 bp, synthetic construct
  source 1..28: mol_type = other DNA
aatcatttaatcctcacaatactaatgg

SEQ ID NO: 27223 - DNA, 28 bp, synthetic construct
  source 1..28: mol_type = other DNA
gaaaatcgtttccattagtattgtgagg

SEQ ID NO: 27224 - DNA, 28 bp, synthetic construct
  source 1..28: mol_type = other DNA
gattttcttccccattatatctgtgagg

SEQ ID NO: 27225 - DNA, 28 bp, synthetic construct
  source 1..28: mol_type = other DNA
attttcttccccattatatctgtgaggg

SEQ ID NO: 27226 - DNA, 28 bp, synthetic construct
  source 1..28: mol_type = other DNA
cctttcatccctcacagatataatgggg

SEQ ID NO: 27227 - DNA, 28 bp, synthetic construct
  source 1..28: mol_type = other DNA
gcctttcatccctcacagatataatggg

SEQ ID NO: 27228 - DNA, 28 bp, synthetic construct
  source 1..28: mol_type = other DNA
agcctttcatccctcacagatataatgg

SEQ ID NO: 27229 - DNA, 28 bp, synthetic construct
  source 1..28: mol_type = other DNA
tctgtgagggatgaaaggctttcaaagg

SEQ ID NO: 27230 - DNA, 28 bp, synthetic construct
  source 1..28: mol_type = other DNA
cacttactagctatgggatctttggtgg

SEQ ID NO: 27231 - DNA, 28 bp, synthetic construct
  source 1..28: mol_type = other DNA
caccaaagatcccatagctagtaagtgg

SEQ ID NO: 27232 - DNA, 28 bp, synthetic construct
  source 1..28: mol_type = other DNA
tgccacttactagctatgggatctttgg

SEQ ID NO: 27233 - DNA, 28 bp, synthetic construct
  source 1..28: mol_type = other DNA
gctgggactgccacttactagctatggg

SEQ ID NO: 27234 - DNA, 28 bp, synthetic construct
  source 1..28: mol_type = other DNA
tgctgggactgccacttactagctatgg

SEQ ID NO: 27235 - DNA, 28 bp, synthetic construct
  source 1..28: mol_type = other DNA
aagtggcagtcccagcattgaaccaagg

SEQ ID NO: 27236 - DNA, 28 bp, synthetic construct
  source 1..28: mol_type = other DNA
atctgaaggaccttggttcaatgctggg

SEQ ID NO: 27237 - DNA, 28 bp, synthetic construct
  source 1..28: mol_type = other DNA
catctgaaggaccttggttcaatgctgg

SEQ ID NO: 27238 - DNA, 28 bp, synthetic construct
  source 1..28: mol_type = other DNA
acagactttggcatctgaaggaccttgg

SEQ ID NO: 27239 - DNA, 28 bp, synthetic construct
  source 1..28: mol_type = other DNA
ctagagcacagactttggcatctgaagg

SEQ ID NO: 27240 - DNA, 28 bp, synthetic construct
  source 1..28: mol_type = other DNA
gtaaacagatctagagcacagactttgg

SEQ ID NO: 27241 - DNA, 28 bp, synthetic construct
  source 1..28: mol_type = other DNA
tagatctgtttacttactgctaattagg

SEQ ID NO: 27242 - DNA, 28 bp, synthetic construct
  source 1..28: mol_type = other DNA
cataaagtgtttgatgcttgcttgtagg

SEQ ID NO: 27243 - DNA, 28 bp, synthetic construct
  source 1..28: mol_type = other DNA
actttatgaagcagaattaatgcaatgg

SEQ ID NO: 27244 - DNA, 28 bp, synthetic construct
  source 1..28: mol_type = other DNA
ttatgaagcagaattaatgcaatggagg

SEQ ID NO: 27245 - DNA, 28 bp, synthetic construct
  source 1..28: mol_type = other DNA
agaattaatgcaatggaggtatctatgg

SEQ ID NO: 27246 - DNA, 28 bp, synthetic construct
  source 1..28: mol_type = other DNA
ttttagtcagaatttgaatatgatgtgg

SEQ ID NO: 27247 - DNA, 28 bp, synthetic construct
  source 1..28: mol_type = other DNA
aaactcacagcatctacctaaattttgg

SEQ ID NO: 27248 - DNA, 28 bp, synthetic construct
  source 1..28: mol_type = other DNA
ttttcaggtagaaactccaaaatttagg

SEQ ID NO: 27249 - DNA, 28 bp, synthetic construct
  source 1..28: mol_type = other DNA
tgaacatgaagaaataaatattttcagg

SEQ ID NO: 27250 - DNA, 28 bp, synthetic construct
  source 1..28: mol_type = other DNA
agaaataaaatttgaggatatttctggg

SEQ ID NO: 27251 - DNA, 28 bp, synthetic construct
  source 1..28: mol_type = other DNA
tagaaataaaatttgaggatatttctgg

SEQ ID NO: 27252 - DNA, 28 bp, synthetic construct
  source 1..28: mol_type = other DNA
acaaacatgatagaaataaaatttgagg

SEQ ID NO: 27253 - DNA, 28 bp, synthetic construct
  source 1..28: mol_type = other DNA
ggctctagaaataattttttttttaagg

SEQ ID NO: 27254 - DNA, 28 bp, synthetic construct
  source 1..28: mol_type = other DNA
agccataaatgttcagcaacaagcctgg

SEQ ID NO: 27255 - DNA, 28 bp, synthetic construct
  source 1..28: mol_type = other DNA
cgccaggcttgttgctgaacatttatgg

SEQ ID NO: 27256 - DNA, 28 bp, synthetic construct
  source 1..28: mol_type = other DNA
atgttcagcaacaagcctggcgcagtgg

SEQ ID NO: 27257 - DNA, 28 bp, synthetic construct
  source 1..28: mol_type = other DNA
gattacaggcgttagccactgcgccagg

SEQ ID NO: 27258 - DNA, 28 bp, synthetic construct
  source 1..28: mol_type = other DNA
gctaacgcctgtaatcccaacactttgg

SEQ ID NO: 27259 - DNA, 28 bp, synthetic construct
  source 1..28: mol_type = other DNA
ctaacgcctgtaatcccaacactttggg

SEQ ID NO: 27260 - DNA, 28 bp, synthetic construct
  source 1..28: mol_type = other DNA
acgcctgtaatcccaacactttgggagg

SEQ ID NO: 27261 - DNA, 28 bp, synthetic construct
  source 1..28: mol_type = other DNA
cggcctcccaaagtgttgggattacagg

SEQ ID NO: 27262 - DNA, 28 bp, synthetic construct
  source 1..28: mol_type = other DNA
gtaatcccaacactttgggaggccgagg

SEQ ID NO: 27263 - DNA, 28 bp, synthetic construct
  source 1..28: mol_type = other DNA
tcccaacactttgggaggccgaggcagg

SEQ ID NO: 27264 - DNA, 28 bp, synthetic construct
  source 1..28: mol_type = other DNA
gcctgcctcggcctcccaaagtgttggg

SEQ ID NO: 27265 - DNA, 28 bp, synthetic construct
  source 1..28: mol_type = other DNA
cgcctgcctcggcctcccaaagtgttgg

SEQ ID NO: 27266 - DNA, 28 bp, synthetic construct
  source 1..28: mol_type = other DNA
caacactttgggaggccgaggcaggcgg

SEQ ID NO: 27267 - DNA, 28 bp, synthetic construct
  source 1..28: mol_type = other DNA
gaggccgaggcaggcggattccctgagg

SEQ ID NO: 27268 - DNA, 28 bp, synthetic construct
  source 1..28: mol_type = other DNA
ctgacctcagggaatccgcctgcctcgg

SEQ ID NO: 27269 - DNA, 28 bp, synthetic construct
  source 1..28: mol_type = other DNA
cgaggcaggcggattccctgaggtcagg

SEQ ID NO: 27270 - DNA, 28 bp, synthetic construct
  source 1..28: mol_type = other DNA
ggctcgtctcaaactcctgacctcaggg

SEQ ID NO: 27271 - DNA, 28 bp, synthetic construct
  source 1..28: mol_type = other DNA
aggctcgtctcaaactcctgacctcagg

SEQ ID NO: 27272 - DNA, 28 bp, synthetic construct
  source 1..28: mol_type = other DNA
tgaggtcaggagtttgagacgagcctgg

SEQ ID NO: 27273 - DNA, 28 bp, synthetic construct
  source 1..28: mol_type = other DNA
gagctgggttttcacaatgttggccagg

SEQ ID NO: 27274 - DNA, 28 bp, synthetic construct
  source 1..28: mol_type = other DNA
taatagagctgggttttcacaatgttgg

SEQ ID NO: 27275 - DNA, 28 bp, synthetic construct
  source 1..28: mol_type = other DNA
aaatttttgtatttttaatagagctggg

SEQ ID NO: 27276 - DNA, 28 bp, synthetic construct
  source 1..28: mol_type = other DNA
caaatttttgtatttttaatagagctgg

SEQ ID NO: 27277 - DNA, 28 bp, synthetic construct
  source 1..28: mol_type = other DNA
cagctctattaaaaatacaaaaatttgg

SEQ ID NO: 27278 - DNA, 28 bp, synthetic construct
  source 1..28: mol_type = other DNA
ctattaaaaatacaaaaatttggccagg

SEQ ID NO: 27279 - DNA, 28 bp, synthetic construct
  source 1..28: mol_type = other DNA
aaaaatacaaaaatttggccaggtgtgg

SEQ ID NO: 27280 - DNA, 28 bp, synthetic construct
  source 1..28: mol_type = other DNA
aatacaaaaatttggccaggtgtggtgg

SEQ ID NO: 27281 - DNA, 28 bp, synthetic construct
  source 1..28: mol_type = other DNA
tattacaggtgtgagccaccacacctgg

SEQ ID NO: 27282 - DNA, 28 bp, synthetic construct
  source 1..28: mol_type = other DNA
gctcacacctgtaataccagcgctttgg

SEQ ID NO: 27283 - DNA, 28 bp, synthetic construct
  source 1..28: mol_type = other DNA
ctcacacctgtaataccagcgctttggg

SEQ ID NO: 27284 - DNA, 28 bp, synthetic construct
  source 1..28: mol_type = other DNA
acacctgtaataccagcgctttgggagg

SEQ ID NO: 27285 - DNA, 28 bp, synthetic construct
  source 1..28: mol_type = other DNA
cggcctcccaaagcgctggtattacagg

SEQ ID NO: 27286 - DNA, 28 bp, synthetic construct
  source 1..28: mol_type = other DNA
gtaataccagcgctttgggaggccgagg

SEQ ID NO: 27287 - DNA, 28 bp, synthetic construct
  source 1..28: mol_type = other DNA
ataccagcgctttgggaggccgaggcgg

SEQ ID NO: 27288 - DNA, 28 bp, synthetic construct
  source 1..28: mol_type = other DNA
taccagcgctttgggaggccgaggcggg

SEQ ID NO: 27289 - DNA, 28 bp, synthetic construct
  source 1..28: mol_type = other DNA
accagcgctttgggaggccgaggcgggg

SEQ ID NO: 27290 - DNA, 28 bp, synthetic construct
  source 1..28: mol_type = other DNA
tccccgcctcggcctcccaaagcgctgg

SEQ ID NO: 27291 - DNA, 28 bp, synthetic construct
  source 1..28: mol_type = other DNA
ggaggccgaggcggggaatcacctgagg

SEQ ID NO: 27292 - DNA, 28 bp, synthetic construct
  source 1..28: mol_type = other DNA
cctgacctcaggtgattccccgcctcgg

SEQ ID NO: 27293 - DNA, 28 bp, synthetic construct
  source 1..28: mol_type = other DNA
aggttggtctcaaactcctgacctcagg

SEQ ID NO: 27294 - DNA, 28 bp, synthetic construct
  source 1..28: mol_type = other DNA
tgaggtcaggagtttgagaccaacctgg

SEQ ID NO: 27295 - DNA, 28 bp, synthetic construct
  source 1..28: mol_type = other DNA
cggggtttcgctttgttggccaggttgg

SEQ ID NO: 27296 - DNA, 28 bp, synthetic construct
  source 1..28: mol_type = other DNA
gagacggggtttcgctttgttggccagg

SEQ ID NO: 27297 - DNA, 28 bp, synthetic construct
  source 1..28: mol_type = other DNA
tagtagagacggggtttcgctttgttgg

SEQ ID NO: 27298 - DNA, 28 bp, synthetic construct
  source 1..28: mol_type = other DNA
attttttgtatatttagtagagacgggg

SEQ ID NO: 27299 - DNA, 28 bp, synthetic construct
  source 1..28: mol_type = other DNA
gattttttgtatatttagtagagacggg

SEQ ID NO: 27300 - DNA, 28 bp, synthetic construct
  source 1..28: mol_type = other DNA
tgattttttgtatatttagtagagacgg

SEQ ID NO: 27301 - DNA, 28 bp, synthetic construct
  source 1..28: mol_type = other DNA
ctactaaatatacaaaaaatcagctagg

SEQ ID NO: 27302 - DNA, 28 bp, synthetic construct
  source 1..28: mol_type = other DNA
aaatatacaaaaaatcagctaggcgtgg

SEQ ID NO: 27303 - DNA, 28 bp, synthetic construct
  source 1..28: mol_type = other DNA
acaaaaaatcagctaggcgtggtgatgg

SEQ ID NO: 27304 - DNA, 28 bp, synthetic construct
  source 1..28: mol_type = other DNA
caaaaaatcagctaggcgtggtgatggg

SEQ ID NO: 27305 - DNA, 28 bp, synthetic construct
  source 1..28: mol_type = other DNA
atgggtgcctgtaatcccagctactcgg

SEQ ID NO: 27306 - DNA, 28 bp, synthetic construct
  source 1..28: mol_type = other DNA
tgggtgcctgtaatcccagctactcggg

SEQ ID NO: 27307 - DNA, 28 bp, synthetic construct
  source 1..28: mol_type = other DNA
gtgcctgtaatcccagctactcgggagg

SEQ ID NO: 27308 - DNA, 28 bp, synthetic construct
  source 1..28: mol_type = other DNA
cagcctcccgagtagctgggattacagg

SEQ ID NO: 27309 - DNA, 28 bp, synthetic construct
  source 1..28: mol_type = other DNA
gtaatcccagctactcgggaggctgagg

SEQ ID NO: 27310 - DNA, 28 bp, synthetic construct
  source 1..28: mol_type = other DNA
ttctgcctcagcctcccgagtagctggg

SEQ ID NO: 27311 - DNA, 28 bp, synthetic construct
  source 1..28: mol_type = other DNA
cttctgcctcagcctcccgagtagctgg

SEQ ID NO: 27312 - DNA, 28 bp, synthetic construct
  source 1..28: mol_type = other DNA
ctgaggcagaagaattgcttgaacccgg

SEQ ID NO: 27313 - DNA, 28 bp, synthetic construct
  source 1..28: mol_type = other DNA
tgaggcagaagaattgcttgaacccggg

SEQ ID NO: 27314 - DNA, 28 bp, synthetic construct
  source 1..28: mol_type = other DNA
ggcagaagaattgcttgaacccgggagg

SEQ ID NO: 27315 - DNA, 28 bp, synthetic construct
  source 1..28: mol_type = other DNA
agaagaattgcttgaacccgggaggtgg

SEQ ID NO: 27316 - DNA, 28 bp, synthetic construct
  source 1..28: mol_type = other DNA
agaattgcttgaacccgggaggtggagg

SEQ ID NO: 27317 - DNA, 28 bp, synthetic construct
  source 1..28: mol_type = other DNA
tggctcactgtaacctccacctcccggg

SEQ ID NO: 27318 - DNA, 28 bp, synthetic construct
  source 1..28: mol_type = other DNA
ttggctcactgtaacctccacctcccgg

SEQ ID NO: 27319 - DNA, 28 bp, synthetic construct
  source 1..28: mol_type = other DNA
agactggagtgcaatggcacgatcttgg

SEQ ID NO: 27320 - DNA, 28 bp, synthetic construct
  source 1..28: mol_type = other DNA
aagatcgtgccattgcactccagtctgg

SEQ ID NO: 27321 - DNA, 28 bp, synthetic construct
  source 1..28: mol_type = other DNA
agatcgtgccattgcactccagtctggg

SEQ ID NO: 27322 - DNA, 28 bp, synthetic construct
  source 1..28: mol_type = other DNA
ctctgtcgcccagactggagtgcaatgg

SEQ ID NO: 27323 - DNA, 28 bp, synthetic construct
  source 1..28: mol_type = other DNA
tagagtctcactctgtcgcccagactgg

SEQ ID NO: 27324 - DNA, 28 bp, synthetic construct
  source 1..28: mol_type = other DNA
aaaaccccaaaaaaatacaaaaattagg

SEQ ID NO: 27325 - DNA, 28 bp, synthetic construct
  source 1..28: mol_type = other DNA
acagcctaatttttgtatttttttgggg

SEQ ID NO: 27326 - DNA, 28 bp, synthetic construct
  source 1..28: mol_type = other DNA
cacagcctaatttttgtatttttttggg

SEQ ID NO: 27327 - DNA, 28 bp, synthetic construct
  source 1..28: mol_type = other DNA
gcacagcctaatttttgtatttttttgg

SEQ ID NO: 27328 - DNA, 28 bp, synthetic construct
  source 1..28: mol_type = other DNA
aaaaatacaaaaattaggctgtgcgcgg

SEQ ID NO: 27329 - DNA, 28 bp, synthetic construct
  source 1..28: mol_type = other DNA
aatacaaaaattaggctgtgcgcggtgg

SEQ ID NO: 27330 - DNA, 28 bp, synthetic construct
  source 1..28: mol_type = other DNA
gctcatgcctgtaatcccagcactttgg

SEQ ID NO: 27331 - DNA, 28 bp, synthetic construct
  source 1..28: mol_type = other DNA
ctcatgcctgtaatcccagcactttggg

SEQ ID NO: 27332 - DNA, 28 bp, synthetic construct
  source 1..28: mol_type = other DNA
atgcctgtaatcccagcactttgggagg

SEQ ID NO: 27333 - DNA, 28 bp, synthetic construct
  source 1..28: mol_type = other DNA
cggcctcccaaagtgctgggattacagg

SEQ ID NO: 27334 - DNA, 28 bp, synthetic construct
  source 1..28: mol_type = other DNA
gtaatcccagcactttgggaggccgagg

SEQ ID NO: 27335 - DNA, 28 bp, synthetic construct
  source 1..28: mol_type = other DNA
atcccagcactttgggaggccgaggtgg

SEQ ID NO: 27336 - DNA, 28 bp, synthetic construct
  source 1..28: mol_type = other DNA
tcccagcactttgggaggccgaggtggg

SEQ ID NO: 27337 - DNA, 28 bp, synthetic construct
  source 1..28: mol_type = other DNA
acccacctcggcctcccaaagtgctggg

SEQ ID NO: 27338 - DNA, 28 bp, synthetic construct
  source 1..28: mol_type = other DNA
cacccacctcggcctcccaaagtgctgg

SEQ ID NO: 27339 - DNA, 28 bp, synthetic construct
  source 1..28: mol_type = other DNA
cagcactttgggaggccgaggtgggtgg

SEQ ID NO: 27340 - DNA, 28 bp, synthetic construct
  source 1..28: mol_type = other DNA
gggaggccgaggtgggtggatcacgagg

SEQ ID NO: 27341 - DNA, 28 bp, synthetic construct
  source 1..28: mol_type = other DNA
gccgaggtgggtggatcacgaggtcagg

SEQ ID NO: 27342 - DNA, 28 bp, synthetic construct
  source 1..28: mol_type = other DNA
tcctgacctcgtgatccacccacctcgg

SEQ ID NO: 27343 - DNA, 28 bp, synthetic construct
  source 1..28: mol_type = other DNA
cgaggtcaggagttcaagaccagcctgg

SEQ ID NO: 27344 - DNA, 28 bp, synthetic construct
  source 1..28: mol_type = other DNA
tcaggagttcaagaccagcctggccagg

SEQ ID NO: 27345 - DNA, 28 bp, synthetic construct
  source 1..28: mol_type = other DNA
gagttcaagaccagcctggccaggatgg

SEQ ID NO: 27346 - DNA, 28 bp, synthetic construct
  source 1..28: mol_type = other DNA
cgaggtttcaccatcctggccaggctgg

SEQ ID NO: 27347 - DNA, 28 bp, synthetic construct
  source 1..28: mol_type = other DNA
gagacgaggtttcaccatcctggccagg

SEQ ID NO: 27348 - DNA, 28 bp, synthetic construct
  source 1..28: mol_type = other DNA
cagtagagacgaggtttcaccatcctgg

SEQ ID NO: 27349 - DNA, 28 bp, synthetic construct
  source 1..28: mol_type = other DNA
aatttttgtagtttcagtagagacgagg

SEQ ID NO: 27350 - DNA, 28 bp, synthetic construct
  source 1..28: mol_type = other DNA
tctactgaaactacaaaaattagccagg

SEQ ID NO: 27351 - DNA, 28 bp, synthetic construct
  source 1..28: mol_type = other DNA
aactacaaaaattagccaggcgcgatgg

SEQ ID NO: 27352 - DNA, 28 bp, synthetic construct
  source 1..28: mol_type = other DNA
acaaaaattagccaggcgcgatggcagg

SEQ ID NO: 27353 - DNA, 28 bp, synthetic construct
  source 1..28: mol_type = other DNA
gattacaggtgcctgccatcgcgcctgg

SEQ ID NO: 27354 - DNA, 28 bp, synthetic construct
  source 1..28: mol_type = other DNA
gcaggcacctgtaatcccagctactcgg

SEQ ID NO: 27355 - DNA, 28 bp, synthetic construct
  source 1..28: mol_type = other DNA
caggcacctgtaatcccagctactcggg

SEQ ID NO: 27356 - DNA, 28 bp, synthetic construct
  source 1..28: mol_type = other DNA
gcacctgtaatcccagctactcgggagg

SEQ ID NO: 27357 - DNA, 28 bp, synthetic construct
  source 1..28: mol_type = other DNA
cagcctcccgagtagctgggattacagg

SEQ ID NO: 27358 - DNA, 28 bp, synthetic construct
  source 1..28: mol_type = other DNA
gtaatcccagctactcgggaggctgagg

SEQ ID NO: 27359 - DNA, 28 bp, synthetic construct
  source 1..28: mol_type = other DNA
tcccagctactcgggaggctgaggcagg

SEQ ID NO: 27360 - DNA, 28 bp, synthetic construct
  source 1..28: mol_type = other DNA
tcctgcctcagcctcccgagtagctggg

SEQ ID NO: 27361 - DNA, 28 bp, synthetic construct
  source 1..28: mol_type = other DNA
ctcctgcctcagcctcccgagtagctgg

SEQ ID NO: 27362 - DNA, 28 bp, synthetic construct
  source 1..28: mol_type = other DNA
ctgaggcaggagaatcgcttgaaaccgg

SEQ ID NO: 27363 - DNA, 28 bp, synthetic construct
  source 1..28: mol_type = other DNA
tgaggcaggagaatcgcttgaaaccggg

SEQ ID NO: 27364 - DNA, 28 bp, synthetic construct
  source 1..28: mol_type = other DNA
ggcaggagaatcgcttgaaaccgggtgg

SEQ ID NO: 27365 - DNA, 28 bp, synthetic construct
  source 1..28: mol_type = other DNA
agaatcgcttgaaaccgggtggctgagg

SEQ ID NO: 27366 - DNA, 28 bp, synthetic construct
  source 1..28: mol_type = other DNA
tcggctcactgcaacctcagccacccgg

SEQ ID NO: 27367 - DNA, 28 bp, synthetic construct
  source 1..28: mol_type = other DNA
gggtggctgaggttgcagtgagccgagg

SEQ ID NO: 27368 - DNA, 28 bp, synthetic construct
  source 1..28: mol_type = other DNA
aggctagagtacagtggtacgacctcgg

SEQ ID NO: 27369 - DNA, 28 bp, synthetic construct
  source 1..28: mol_type = other DNA
gaggtcgtaccactgtactctagcctgg

SEQ ID NO: 27370 - DNA, 28 bp, synthetic construct
  source 1..28: mol_type = other DNA
aggtcgtaccactgtactctagcctggg

SEQ ID NO: 27371 - DNA, 28 bp, synthetic construct
  source 1..28: mol_type = other DNA
ctctgtcacccaggctagagtacagtgg

SEQ ID NO: 27372 - DNA, 28 bp, synthetic construct
  source 1..28: mol_type = other DNA
gtactctagcctgggtgacagagtgagg

SEQ ID NO: 27373 - DNA, 28 bp, synthetic construct
  source 1..28: mol_type = other DNA
ctctagcctgggtgacagagtgaggcgg

SEQ ID NO: 27374 - DNA, 28 bp, synthetic construct
  source 1..28: mol_type = other DNA
ctttttccgcctcactctgtcacccagg

SEQ ID NO: 27375 - DNA, 28 bp, synthetic construct
  source 1..28: mol_type = other DNA
aaacaaaacaaaaattagccaagcctgg

SEQ ID NO: 27376 - DNA, 28 bp, synthetic construct
  source 1..28: mol_type = other DNA
gattacaggcgctcgtcaccaggcttgg

SEQ ID NO: 27377 - DNA, 28 bp, synthetic construct
  source 1..28: mol_type = other DNA
gctgggattacaggcgctcgtcaccagg

SEQ ID NO: 27378 - DNA, 28 bp, synthetic construct
  source 1..28: mol_type = other DNA
cgagcgcctgtaatcccagctactcagg

SEQ ID NO: 27379 - DNA, 28 bp, synthetic construct
  source 1..28: mol_type = other DNA
gcgcctgtaatcccagctactcaggagg

SEQ ID NO: 27380 - DNA, 28 bp, synthetic construct
  source 1..28: mol_type = other DNA
cagcctcctgagtagctgggattacagg

SEQ ID NO: 27381 - DNA, 28 bp, synthetic construct
  source 1..28: mol_type = other DNA
gtaatcccagctactcaggaggctgagg

SEQ ID NO: 27382 - DNA, 28 bp, synthetic construct
  source 1..28: mol_type = other DNA
tcatgcctcagcctcctgagtagctggg

SEQ ID NO: 27383 - DNA, 28 bp, synthetic construct
  source 1..28: mol_type = other DNA
ctcatgcctcagcctcctgagtagctgg

SEQ ID NO: 27384 - DNA, 28 bp, synthetic construct
  source 1..28: mol_type = other DNA
tgaggcatgagaatcgcttaaacccagg

SEQ ID NO: 27385 - DNA, 28 bp, synthetic construct
  source 1..28: mol_type = other DNA
ggcatgagaatcgcttaaacccaggagg

SEQ ID NO: 27386 - DNA, 28 bp, synthetic construct
  source 1..28: mol_type = other DNA
atgagaatcgcttaaacccaggaggcgg

SEQ ID NO: 27387 - DNA, 28 bp, synthetic construct
  source 1..28: mol_type = other DNA
agaatcgcttaaacccaggaggcggagg

SEQ ID NO: 27388 - DNA, 28 bp, synthetic construct
  source 1..28: mol_type = other DNA
cagctcactgcagcctccgcctcctggg

SEQ ID NO: 27389 - DNA, 28 bp, synthetic construct
  source 1..28: mol_type = other DNA
tcagctcactgcagcctccgcctcctgg

SEQ ID NO: 27390 - DNA, 28 bp, synthetic construct
  source 1..28: mol_type = other DNA
agattgcgccactgcaacaaccagcagg

SEQ ID NO: 27391 - DNA, 28 bp, synthetic construct
  source 1..28: mol_type = other DNA
gccactgcaacaaccagcaggcctgagg

SEQ ID NO: 27392 - DNA, 28 bp, synthetic construct
  source 1..28: mol_type = other DNA
gcctcaggcctgctggttgttgcagtgg

SEQ ID NO: 27393 - DNA, 28 bp, synthetic construct
  source 1..28: mol_type = other DNA
aaccagcaggcctgaggctcatcctagg

SEQ ID NO: 27394 - DNA, 28 bp, synthetic construct
  source 1..28: mol_type = other DNA
aggctgggacaaatagttttcagctggg

SEQ ID NO: 27395 - DNA, 28 bp, synthetic construct
  source 1..28: mol_type = other DNA
gaggctgggacaaatagttttcagctgg

SEQ ID NO: 27396 - DNA, 28 bp, synthetic construct
  source 1..28: mol_type = other DNA
tgaaaactatttgtcccagcctctaagg

SEQ ID NO: 27397 - DNA, 28 bp, synthetic construct
  source 1..28: mol_type = other DNA
agactgtcacaggaccttagaggctggg

SEQ ID NO: 27398 - DNA, 28 bp, synthetic construct
  source 1..28: mol_type = other DNA
cagactgtcacaggaccttagaggctgg

SEQ ID NO: 27399 - DNA, 28 bp, synthetic construct
  source 1..28: mol_type = other DNA
cagcctctaaggtcctgtgacagtctgg

SEQ ID NO: 27400 - DNA, 28 bp, synthetic construct
  source 1..28: mol_type = other DNA
tggccagactgtcacaggaccttagagg

SEQ ID NO: 27401 - DNA, 28 bp, synthetic construct
  source 1..28: mol_type = other DNA
taaggtcctgtgacagtctggccaatgg

SEQ ID NO: 27402 - DNA, 28 bp, synthetic construct
  source 1..28: mol_type = other DNA
aaggtcctgtgacagtctggccaatggg

SEQ ID NO: 27403 - DNA, 28 bp, synthetic construct
  source 1..28: mol_type = other DNA
ttattcccattggccagactgtcacagg

SEQ ID NO: 27404 - DNA, 28 bp, synthetic construct
  source 1..28: mol_type = other DNA
gccaatgggaataagcagaaaccactgg

SEQ ID NO: 27405 - DNA, 28 bp, synthetic construct
  source 1..28: mol_type = other DNA
ccaatgggaataagcagaaaccactggg

SEQ ID NO: 27406 - DNA, 28 bp, synthetic construct
  source 1..28: mol_type = other DNA
tgggaataagcagaaaccactgggttgg

SEQ ID NO: 27407 - DNA, 28 bp, synthetic construct
  source 1..28: mol_type = other DNA
gggaataagcagaaaccactgggttggg

SEQ ID NO: 27408 - DNA, 28 bp, synthetic construct
  source 1..28: mol_type = other DNA
ggaataagcagaaaccactgggttgggg

SEQ ID NO: 27409 - DNA, 28 bp, synthetic construct
  source 1..28: mol_type = other DNA
gcagaaaccactgggttggggctgcagg

SEQ ID NO: 27410 - DNA, 28 bp, synthetic construct
  source 1..28: mol_type = other DNA
gcgttttcctgcagccccaacccagtgg

SEQ ID NO: 27411 - DNA, 28 bp, synthetic construct
  source 1..28: mol_type = other DNA
gggctgcaggaaaacgctgacaaagagg

SEQ ID NO: 27412 - DNA, 28 bp, synthetic construct
  source 1..28: mol_type = other DNA
gcaggaaaacgctgacaaagaggactgg

SEQ ID NO: 27413 - DNA, 28 bp, synthetic construct
  source 1..28: mol_type = other DNA
aacgctgacaaagaggactggctccagg

SEQ ID NO: 27414 - DNA, 28 bp, synthetic construct
  source 1..28: mol_type = other DNA
aggcagcagtgaggacaaaggtacctgg

SEQ ID NO: 27415 - DNA, 28 bp, synthetic construct
  source 1..28: mol_type = other DNA
acctttgtcctcactgctgcctgcctgg

SEQ ID NO: 27416 - DNA, 28 bp, synthetic construct
  source 1..28: mol_type = other DNA
tccaggcaggcagcagtgaggacaaagg

SEQ ID NO: 27417 - DNA, 28 bp, synthetic construct
  source 1..28: mol_type = other DNA
cctatgttccaggcaggcagcagtgagg

SEQ ID NO: 27418 - DNA, 28 bp, synthetic construct
  source 1..28: mol_type = other DNA
cggcagcaaaacctatgttccaggcagg

SEQ ID NO: 27419 - DNA, 28 bp, synthetic construct
  source 1..28: mol_type = other DNA
ctgcctggaacataggttttgctgccgg

SEQ ID NO: 27420 - DNA, 28 bp, synthetic construct
  source 1..28: mol_type = other DNA
tgcctggaacataggttttgctgccggg

SEQ ID NO: 27421 - DNA, 28 bp, synthetic construct
  source 1..28: mol_type = other DNA
gcctggaacataggttttgctgccgggg

SEQ ID NO: 27422 - DNA, 28 bp, synthetic construct
  source 1..28: mol_type = other DNA
cctggaacataggttttgctgccggggg

SEQ ID NO: 27423 - DNA, 28 bp, synthetic construct
  source 1..28: mol_type = other DNA
aacataggttttgctgccgggggtgagg

SEQ ID NO: 27424 - DNA, 28 bp, synthetic construct
  source 1..28: mol_type = other DNA
acataggttttgctgccgggggtgaggg

SEQ ID NO: 27425 - DNA, 28 bp, synthetic construct
  source 1..28: mol_type = other DNA
cataggttttgctgccgggggtgagggg

SEQ ID NO: 27426 - DNA, 28 bp, synthetic construct
  source 1..28: mol_type = other DNA
aggttttgctgccgggggtgaggggtgg

SEQ ID NO: 27427 - DNA, 28 bp, synthetic construct
  source 1..28: mol_type = other DNA
ggttttgctgccgggggtgaggggtggg

SEQ ID NO: 27428 - DNA, 28 bp, synthetic construct
  source 1..28: mol_type = other DNA
gctgccgggggtgaggggtgggaacagg

SEQ ID NO: 27429 - DNA, 28 bp, synthetic construct
  source 1..28: mol_type = other DNA
cctgcctgttcccacccctcacccccgg

SEQ ID NO: 27430 - DNA, 28 bp, synthetic construct
  source 1..28: mol_type = other DNA
aggcaggagccatcctgtgacagcaagg

SEQ ID NO: 27431 - DNA, 28 bp, synthetic construct
  source 1..28: mol_type = other DNA
tgcattttaccttgctgtcacaggatgg

SEQ ID NO: 27432 - DNA, 28 bp, synthetic construct
  source 1..28: mol_type = other DNA
aatgtgcattttaccttgctgtcacagg

SEQ ID NO: 27433 - DNA, 28 bp, synthetic construct
  source 1..28: mol_type = other DNA
aaggtaaaatgcacattcctaagaaagg

SEQ ID NO: 27434 - DNA, 28 bp, synthetic construct
  source 1..28: mol_type = other DNA
gctggtatttctgcttacctttcttagg

SEQ ID NO: 27435 - DNA, 28 bp, synthetic construct
  source 1..28: mol_type = other DNA
aagcagaaataccagcattgagtcatgg

SEQ ID NO: 27436 - DNA, 28 bp, synthetic construct
  source 1..28: mol_type = other DNA
agcagaaataccagcattgagtcatggg

SEQ ID NO: 27437 - DNA, 28 bp, synthetic construct
  source 1..28: mol_type = other DNA
cttgatgtcacccatgactcaatgctgg

SEQ ID NO: 27438 - DNA, 28 bp, synthetic construct
  source 1..28: mol_type = other DNA
gagagagacttaagggctgttactgtgg

SEQ ID NO: 27439 - DNA, 28 bp, synthetic construct
  source 1..28: mol_type = other DNA
atatgaattctggagagagacttaaggg

SEQ ID NO: 27440 - DNA, 28 bp, synthetic construct
  source 1..28: mol_type = other DNA
gatatgaattctggagagagacttaagg

SEQ ID NO: 27441 - DNA, 28 bp, synthetic construct
  source 1..28: mol_type = other DNA
tatgtttctcatgtgatatgaattctgg

SEQ ID NO: 27442 - DNA, 28 bp, synthetic construct
  source 1..28: mol_type = other DNA
atatcacatgagaaacataaactcctgg

SEQ ID NO: 27443 - DNA, 28 bp, synthetic construct
  source 1..28: mol_type = other DNA
agctattcactaggtctatcacataagg

SEQ ID NO: 27444 - DNA, 28 bp, synthetic construct
  source 1..28: mol_type = other DNA
ggcaaagccagctctacttgtgttctgg

SEQ ID NO: 27445 - DNA, 28 bp, synthetic construct
  source 1..28: mol_type = other DNA
tttagctccagaacacaagtagagctgg

SEQ ID NO: 27446 - DNA, 28 bp, synthetic construct
  source 1..28: mol_type = other DNA
attcggaatctgtgatagaaggggaagg

SEQ ID NO: 27447 - DNA, 28 bp, synthetic construct
  source 1..28: mol_type = other DNA
aaacattcggaatctgtgatagaagggg

SEQ ID NO: 27448 - DNA, 28 bp, synthetic construct
  source 1..28: mol_type = other DNA
gaaacattcggaatctgtgatagaaggg

SEQ ID NO: 27449 - DNA, 28 bp, synthetic construct
  source 1..28: mol_type = other DNA
ggaaacattcggaatctgtgatagaagg

SEQ ID NO: 27450 - DNA, 28 bp, synthetic construct
  source 1..28: mol_type = other DNA
tatcacagattccgaatgtttcctctgg

SEQ ID NO: 27451 - DNA, 28 bp, synthetic construct
  source 1..28: mol_type = other DNA
atcacagattccgaatgtttcctctggg

SEQ ID NO: 27452 - DNA, 28 bp, synthetic construct
  source 1..28: mol_type = other DNA
ttccgaatgtttcctctgggcacagtgg

SEQ ID NO: 27453 - DNA, 28 bp, synthetic construct
  source 1..28: mol_type = other DNA
agccactgtgcccagaggaaacattcgg

SEQ ID NO: 27454 - DNA, 28 bp, synthetic construct
  source 1..28: mol_type = other DNA
tgcaggtgtgagccactgtgcccagagg

SEQ ID NO: 27455 - DNA, 28 bp, synthetic construct
  source 1..28: mol_type = other DNA
gcacagtggctcacacctgcaatcctgg

SEQ ID NO: 27456 - DNA, 28 bp, synthetic construct
  source 1..28: mol_type = other DNA
gctcacacctgcaatcctggtgctttgg

SEQ ID NO: 27457 - DNA, 28 bp, synthetic construct
  source 1..28: mol_type = other DNA
ctcacacctgcaatcctggtgctttggg

SEQ ID NO: 27458 - DNA, 28 bp, synthetic construct
  source 1..28: mol_type = other DNA
acacctgcaatcctggtgctttgggagg

SEQ ID NO: 27459 - DNA, 28 bp, synthetic construct
  source 1..28: mol_type = other DNA
gggcctcccaaagcaccaggattgcagg

SEQ ID NO: 27460 - DNA, 28 bp, synthetic construct
  source 1..28: mol_type = other DNA
atcctggtgctttgggaggcccagctgg

SEQ ID NO: 27461 - DNA, 28 bp, synthetic construct
  source 1..28: mol_type = other DNA
ttccagctgggcctcccaaagcaccagg

SEQ ID NO: 27462 - DNA, 28 bp, synthetic construct
  source 1..28: mol_type = other DNA
tggtgctttgggaggcccagctggaagg

SEQ ID NO: 27463 - DNA, 28 bp, synthetic construct
  source 1..28: mol_type = other DNA
gaggcccagctggaaggatcacttgagg

SEQ ID NO: 27464 - DNA, 28 bp, synthetic construct
  source 1..28: mol_type = other DNA
aggcccagctggaaggatcacttgaggg

SEQ ID NO: 27465 - DNA, 28 bp, synthetic construct
  source 1..28: mol_type = other DNA
ctaccctcaagtgatccttccagctggg

SEQ ID NO: 27466 - DNA, 28 bp, synthetic construct
  source 1..28: mol_type = other DNA
ccagctggaaggatcacttgagggtagg

SEQ ID NO: 27467 - DNA, 28 bp, synthetic construct
  source 1..28: mol_type = other DNA
tgagggtaggagtttgagaccagcctgg

SEQ ID NO: 27468 - DNA, 28 bp, synthetic construct
  source 1..28: mol_type = other DNA
gagggtaggagtttgagaccagcctggg

SEQ ID NO: 27469 - DNA, 28 bp, synthetic construct
  source 1..28: mol_type = other DNA
tggtgtcttactgtgttgcccaggctgg

SEQ ID NO: 27470 - DNA, 28 bp, synthetic construct
  source 1..28: mol_type = other DNA
gagctggtgtcttactgtgttgcccagg

SEQ ID NO: 27471 - DNA, 28 bp, synthetic construct
  source 1..28: mol_type = other DNA
aattaaaaaaattttttggcagagctgg

SEQ ID NO: 27472 - DNA, 28 bp, synthetic construct
  source 1..28: mol_type = other DNA
ctgccaaaaaatttttttaattagctgg

SEQ ID NO: 27473 - DNA, 28 bp, synthetic construct
  source 1..28: mol_type = other DNA
tgccaaaaaatttttttaattagctggg

SEQ ID NO: 27474 - DNA, 28 bp, synthetic construct
  source 1..28: mol_type = other DNA
gccaaaaaatttttttaattagctgggg

SEQ ID NO: 27475 - DNA, 28 bp, synthetic construct
  source 1..28: mol_type = other DNA
tccccagctaattaaaaaaattttttgg

SEQ ID NO: 27476 - DNA, 28 bp, synthetic construct
  source 1..28: mol_type = other DNA
aaaaatttttttaattagctggggatgg

SEQ ID NO: 27477 - DNA, 28 bp, synthetic construct
  source 1..28: mol_type = other DNA
aatttttttaattagctggggatggtgg

SEQ ID NO: 27478 - DNA, 28 bp, synthetic construct
  source 1..28: mol_type = other DNA
gtgtgcatgtgtagttccagcttcttgg

SEQ ID NO: 27479 - DNA, 28 bp, synthetic construct
  source 1..28: mol_type = other DNA
tgtgcatgtgtagttccagcttcttggg

SEQ ID NO: 27480 - DNA, 28 bp, synthetic construct
  source 1..28: mol_type = other DNA
gcatgtgtagttccagcttcttgggagg

SEQ ID NO: 27481 - DNA, 28 bp, synthetic construct
  source 1..28: mol_type = other DNA
ttccagcttcttgggaggcagagacagg

SEQ ID NO: 27482 - DNA, 28 bp, synthetic construct
  source 1..28: mol_type = other DNA
ctcctgtctctgcctcccaagaagctgg

SEQ ID NO: 27483 - DNA, 28 bp, synthetic construct
  source 1..28: mol_type = other DNA
cagcttcttgggaggcagagacaggagg

SEQ ID NO: 27484 - DNA, 28 bp, synthetic construct
  source 1..28: mol_type = other DNA
agagacaggaggattgcttgaactcagg

SEQ ID NO: 27485 - DNA, 28 bp, synthetic construct
  source 1..28: mol_type = other DNA
agcatcctgctactgcactctagcctgg

SEQ ID NO: 27486 - DNA, 28 bp, synthetic construct
  source 1..28: mol_type = other DNA
gcatcctgctactgcactctagcctggg

SEQ ID NO: 27487 - DNA, 28 bp, synthetic construct
  source 1..28: mol_type = other DNA
gttgcccaggctagagtgcagtagcagg

SEQ ID NO: 27488 - DNA, 28 bp, synthetic construct
  source 1..28: mol_type = other DNA
gcactctagcctgggcaacagagtaagg

SEQ ID NO: 27489 - DNA, 28 bp, synthetic construct
  source 1..28: mol_type = other DNA
ttaacagggccttactctgttgcccagg

SEQ ID NO: 27490 - DNA, 28 bp, synthetic construct
  source 1..28: mol_type = other DNA
atgggaaacttttttttttttaacaggg

SEQ ID NO: 27491 - DNA, 28 bp, synthetic construct
  source 1..28: mol_type = other DNA
gatgggaaacttttttttttttaacagg

SEQ ID NO: 27492 - DNA, 28 bp, synthetic construct
  source 1..28: mol_type = other DNA
tggattaacaggtttcactgctgatggg

SEQ ID NO: 27493 - DNA, 28 bp, synthetic construct
  source 1..28: mol_type = other DNA
ttggattaacaggtttcactgctgatgg

SEQ ID NO: 27494 - DNA, 28 bp, synthetic construct
  source 1..28: mol_type = other DNA
atcagcagtgaaacctgttaatccaagg

SEQ ID NO: 27495 - DNA, 28 bp, synthetic construct
  source 1..28: mol_type = other DNA
tgaggctgagaaaccttggattaacagg

SEQ ID NO: 27496 - DNA, 28 bp, synthetic construct
  source 1..28: mol_type = other DNA
cagtagtgctgaggctgagaaaccttgg

SEQ ID NO: 27497 - DNA, 28 bp, synthetic construct
  source 1..28: mol_type = other DNA
tcagcctcagcactactgacattttagg

SEQ ID NO: 27498 - DNA, 28 bp, synthetic construct
  source 1..28: mol_type = other DNA
ctagcctaaaatgtcagtagtgctgagg

SEQ ID NO: 27499 - DNA, 28 bp, synthetic construct
  source 1..28: mol_type = other DNA
acattttaggctagctaattttttttgg

SEQ ID NO: 27500 - DNA, 28 bp, synthetic construct
  source 1..28: mol_type = other DNA
cattttaggctagctaattttttttggg

SEQ ID NO: 27501 - DNA, 28 bp, synthetic construct
  source 1..28: mol_type = other DNA
attttaggctagctaattttttttgggg

SEQ ID NO: 27502 - DNA, 28 bp, synthetic construct
  source 1..28: mol_type = other DNA
ttttaggctagctaattttttttggggg

SEQ ID NO: 27503 - DNA, 28 bp, synthetic construct
  source 1..28: mol_type = other DNA
tttaggctagctaattttttttgggggg

SEQ ID NO: 27504 - DNA, 28 bp, synthetic construct
  source 1..28: mol_type = other DNA
ttaggctagctaattttttttggggggg

SEQ ID NO: 27505 - DNA, 28 bp, synthetic construct
  source 1..28: mol_type = other DNA
taggctagctaattttttttgggggggg

SEQ ID NO: 27506 - DNA, 28 bp, synthetic construct
  source 1..28: mol_type = other DNA
aggctagctaattttttttggggggggg

SEQ ID NO: 27507 - DNA, 28 bp, synthetic construct
  source 1..28: mol_type = other DNA
ggctagctaattttttttgggggggggg

SEQ ID NO: 27508 - DNA, 28 bp, synthetic construct
  source 1..28: mol_type = other DNA
gctagctaattttttttggggggggggg

SEQ ID NO: 27509 - DNA, 28 bp, synthetic construct
  source 1..28: mol_type = other DNA
ctagctaattttttttgggggggggggg

SEQ ID NO: 27510 - DNA, 28 bp, synthetic construct
  source 1..28: mol_type = other DNA
tagctaattttttttggggggggggggg

SEQ ID NO: 27511 - DNA, 28 bp, synthetic construct
  source 1..28: mol_type = other DNA
ttttttttgggggggggggggcaagtgg

SEQ ID NO: 27512 - DNA, 28 bp, synthetic construct
  source 1..28: mol_type = other DNA
tttttttgggggggggggggcaagtggg

SEQ ID NO: 27513 - DNA, 28 bp, synthetic construct
  source 1..28: mol_type = other DNA
ttttttgggggggggggggcaagtgggg

SEQ ID NO: 27514 - DNA, 28 bp, synthetic construct
  source 1..28: mol_type = other DNA
aagtggggactgtcttgtgtattgcagg

SEQ ID NO: 27515 - DNA, 28 bp, synthetic construct
  source 1..28: mol_type = other DNA
gcaggatgtttagcagcagcatccctgg

SEQ ID NO: 27516 - DNA, 28 bp, synthetic construct
  source 1..28: mol_type = other DNA
actgacatctaatgggtagaggccaggg

SEQ ID NO: 27517 - DNA, 28 bp, synthetic construct
  source 1..28: mol_type = other DNA
cactgacatctaatgggtagaggccagg

SEQ ID NO: 27518 - DNA, 28 bp, synthetic construct
  source 1..28: mol_type = other DNA
ctggcctctacccattagatgtcagtgg

SEQ ID NO: 27519 - DNA, 28 bp, synthetic construct
  source 1..28: mol_type = other DNA
ggtgccactgacatctaatgggtagagg

SEQ ID NO: 27520 - DNA, 28 bp, synthetic construct
  source 1..28: mol_type = other DNA
gggaggggtgccactgacatctaatggg

SEQ ID NO: 27521 - DNA, 28 bp, synthetic construct
  source 1..28: mol_type = other DNA
agggaggggtgccactgacatctaatgg

SEQ ID NO: 27522 - DNA, 28 bp, synthetic construct
  source 1..28: mol_type = other DNA
ttttggttgttacagatgcagggagggg

SEQ ID NO: 27523 - DNA, 28 bp, synthetic construct
  source 1..28: mol_type = other DNA
gttttggttgttacagatgcagggaggg

SEQ ID NO: 27524 - DNA, 28 bp, synthetic construct
  source 1..28: mol_type = other DNA
agttttggttgttacagatgcagggagg

SEQ ID NO: 27525 - DNA, 28 bp, synthetic construct
  source 1..28: mol_type = other DNA
gagagttttggttgttacagatgcaggg

SEQ ID NO: 27526 - DNA, 28 bp, synthetic construct
  source 1..28: mol_type = other DNA
agagagttttggttgttacagatgcagg

SEQ ID NO: 27527 - DNA, 28 bp, synthetic construct
  source 1..28: mol_type = other DNA
atctgtaacaaccaaaactctctccagg

SEQ ID NO: 27528 - DNA, 28 bp, synthetic construct
  source 1..28: mol_type = other DNA
atttggcaatgcctggagagagttttgg

SEQ ID NO: 27529 - DNA, 28 bp, synthetic construct
  source 1..28: mol_type = other DNA
ctgtggaaggacatttggcaatgcctgg

SEQ ID NO: 27530 - DNA, 28 bp, synthetic construct
  source 1..28: mol_type = other DNA
atggattttgctgtggaaggacatttgg

SEQ ID NO: 27531 - DNA, 28 bp, synthetic construct
  source 1..28: mol_type = other DNA
tgttcatgatggattttgctgtggaagg

SEQ ID NO: 27532 - DNA, 28 bp, synthetic construct
  source 1..28: mol_type = other DNA
gatatgttcatgatggattttgctgtgg

SEQ ID NO: 27533 - DNA, 28 bp, synthetic construct
  source 1..28: mol_type = other DNA
gtgttggtgggggatatgttcatgatgg

SEQ ID NO: 27534 - DNA, 28 bp, synthetic construct
  source 1..28: mol_type = other DNA
cggtggttctctactgtgttggtggggg

SEQ ID NO: 27535 - DNA, 28 bp, synthetic construct
  source 1..28: mol_type = other DNA
acggtggttctctactgtgttggtgggg

SEQ ID NO: 27536 - DNA, 28 bp, synthetic construct
  source 1..28: mol_type = other DNA
aacggtggttctctactgtgttggtggg

SEQ ID NO: 27537 - DNA, 28 bp, synthetic construct
  source 1..28: mol_type = other DNA
gaacggtggttctctactgtgttggtgg

SEQ ID NO: 27538 - DNA, 28 bp, synthetic construct
  source 1..28: mol_type = other DNA
tgagaacggtggttctctactgtgttgg

SEQ ID NO: 27539 - DNA, 28 bp, synthetic construct
  source 1..28: mol_type = other DNA
ctagtttggtattaaatgagaacggtgg

SEQ ID NO: 27540 - DNA, 28 bp, synthetic construct
  source 1..28: mol_type = other DNA
gatctagtttggtattaaatgagaacgg

SEQ ID NO: 27541 - DNA, 28 bp, synthetic construct
  source 1..28: mol_type = other DNA
catttaataccaaactagatctaaatgg

SEQ ID NO: 27542 - DNA, 28 bp, synthetic construct
  source 1..28: mol_type = other DNA
aataccaaactagatctaaatggcaagg

SEQ ID NO: 27543 - DNA, 28 bp, synthetic construct
  source 1..28: mol_type = other DNA
agatccttgccatttagatctagtttgg

SEQ ID NO: 27544 - DNA, 28 bp, synthetic construct
  source 1..28: mol_type = other DNA
taaaaataattagatttaaaatttttgg

SEQ ID NO: 27545 - DNA, 28 bp, synthetic construct
  source 1..28: mol_type = other DNA
atatgatttttgctcaaaaaaagcaagg

SEQ ID NO: 27546 - DNA, 28 bp, synthetic construct
  source 1..28: mol_type = other DNA
agtcactagttaatttctttcttagtgg

SEQ ID NO: 27547 - DNA, 28 bp, synthetic construct
  source 1..28: mol_type = other DNA
tcttagtggcaatgatccaaaatgtagg

SEQ ID NO: 27548 - DNA, 28 bp, synthetic construct
  source 1..28: mol_type = other DNA
tttgtgctatgagttgcctacattttgg

SEQ ID NO: 27549 - DNA, 28 bp, synthetic construct
  source 1..28: mol_type = other DNA
tttcacagttacttataatgttgaaagg

SEQ ID NO: 27550 - DNA, 28 bp, synthetic construct
  source 1..28: mol_type = other DNA
aaatgtctaatgacaaagaaaagactgg

SEQ ID NO: 27551 - DNA, 28 bp, synthetic construct
  source 1..28: mol_type = other DNA
aagaaaagactggttgaataaatcgtgg

SEQ ID NO: 27552 - DNA, 28 bp, synthetic construct
  source 1..28: mol_type = other DNA
ttaaaagagctgcatgatattcacttgg

SEQ ID NO: 27553 - DNA, 28 bp, synthetic construct
  source 1..28: mol_type = other DNA
aatatcatgcagctcttttaaaaacagg

SEQ ID NO: 27554 - DNA, 28 bp, synthetic construct
  source 1..28: mol_type = other DNA
ttaaaaacaggccctcataccaaattgg

SEQ ID NO: 27555 - DNA, 28 bp, synthetic construct
  source 1..28: mol_type = other DNA
ttatgctactgccaatttggtatgaggg

SEQ ID NO: 27556 - DNA, 28 bp, synthetic construct
  source 1..28: mol_type = other DNA
tttatgctactgccaatttggtatgagg

SEQ ID NO: 27557 - DNA, 28 bp, synthetic construct
  source 1..28: mol_type = other DNA
ttgtgagtttatgctactgccaatttgg

SEQ ID NO: 27558 - DNA, 28 bp, synthetic construct
  source 1..28: mol_type = other DNA
gcagtagcataaactcacaatctcttgg

SEQ ID NO: 27559 - DNA, 28 bp, synthetic construct
  source 1..28: mol_type = other DNA
gaaagataatatatgacataaacaaagg

SEQ ID NO: 27560 - DNA, 28 bp, synthetic construct
  source 1..28: mol_type = other DNA
aacaaaggaaaaacaaatcagtaaatgg

SEQ ID NO: 27561 - DNA, 28 bp, synthetic construct
  source 1..28: mol_type = other DNA
tgagctattattaatacacgctatttgg

SEQ ID NO: 27562 - DNA, 28 bp, synthetic construct
  source 1..28: mol_type = other DNA
tttcaaatacagctaaggagctaagtgg

SEQ ID NO: 27563 - DNA, 28 bp, synthetic construct
  source 1..28: mol_type = other DNA
tgtgtttaagtttcaaatacagctaagg

SEQ ID NO: 27564 - DNA, 28 bp, synthetic construct
  source 1..28: mol_type = other DNA
aaaaggtggtgtgtggtcttaatgtagg

SEQ ID NO: 27565 - DNA, 28 bp, synthetic construct
  source 1..28: mol_type = other DNA
gactactttggaaaaaggtggtgtgtgg

SEQ ID NO: 27566 - DNA, 28 bp, synthetic construct
  source 1..28: mol_type = other DNA
aaaattagactactttggaaaaaggtgg

SEQ ID NO: 27567 - DNA, 28 bp, synthetic construct
  source 1..28: mol_type = other DNA
cctttttccaaagtagtctaatttttgg

SEQ ID NO: 27568 - DNA, 28 bp, synthetic construct
  source 1..28: mol_type = other DNA
taatgttccaaaaattagactactttgg

SEQ ID NO: 27569 - DNA, 28 bp, synthetic construct
  source 1..28: mol_type = other DNA
gtctaatttttggaacattatgaaatgg

SEQ ID NO: 27570 - DNA, 28 bp, synthetic construct
  source 1..28: mol_type = other DNA
ttatgaaatggtccattctgatcaatgg

SEQ ID NO: 27571 - DNA, 28 bp, synthetic construct
  source 1..28: mol_type = other DNA
taagctataaggccattgatcagaatgg

SEQ ID NO: 27572 - DNA, 28 bp, synthetic construct
  source 1..28: mol_type = other DNA
tctttgggcatggagataagctataagg

SEQ ID NO: 27573 - DNA, 28 bp, synthetic construct
  source 1..28: mol_type = other DNA
gtttacaatttaaaatctttgggcatgg

SEQ ID NO: 27574 - DNA, 28 bp, synthetic construct
  source 1..28: mol_type = other DNA
ggtatgtttacaatttaaaatctttggg

SEQ ID NO: 27575 - DNA, 28 bp, synthetic construct
  source 1..28: mol_type = other DNA
aggtatgtttacaatttaaaatctttgg

SEQ ID NO: 27576 - DNA, 28 bp, synthetic construct
  source 1..28: mol_type = other DNA
tgtctcaaaaaaaaaaaaggaaagtagg

SEQ ID NO: 27577 - DNA, 28 bp, synthetic construct
  source 1..28: mol_type = other DNA
caagactctgtctcaaaaaaaaaaaagg

SEQ ID NO: 27578 - DNA, 28 bp, synthetic construct
  source 1..28: mol_type = other DNA
tgagacagagtcttgctctgttgccagg

SEQ ID NO: 27579 - DNA, 28 bp, synthetic construct
  source 1..28: mol_type = other DNA
cagagtcttgctctgttgccaggctagg

SEQ ID NO: 27580 - DNA, 28 bp, synthetic construct
  source 1..28: mol_type = other DNA
agagtcttgctctgttgccaggctaggg

SEQ ID NO: 27581 - DNA, 28 bp, synthetic construct
  source 1..28: mol_type = other DNA
gctctgttgccaggctagggtgcagtgg

SEQ ID NO: 27582 - DNA, 28 bp, synthetic construct
  source 1..28: mol_type = other DNA
gagattgcaccactgcaccctagcctgg

SEQ ID NO: 27583 - DNA, 28 bp, synthetic construct
  source 1..28: mol_type = other DNA
aggctagggtgcagtggtgcaatctcgg

SEQ ID NO: 27584 - DNA, 28 bp, synthetic construct
  source 1..28: mol_type = other DNA
tcggctcactgcaacctcagcctccagg

SEQ ID NO: 27585 - DNA, 28 bp, synthetic construct
  source 1..28: mol_type = other DNA
cggctcactgcaacctcagcctccaggg

SEQ ID NO: 27586 - DNA, 28 bp, synthetic construct
  source 1..28: mol_type = other DNA
agaatcgatttaaccctggaggctgagg

SEQ ID NO: 27587 - DNA, 28 bp, synthetic construct
  source 1..28: mol_type = other DNA
ggcaggagaatcgatttaaccctggagg

SEQ ID NO: 27588 - DNA, 28 bp, synthetic construct
  source 1..28: mol_type = other DNA
tgaggcaggagaatcgatttaaccctgg

SEQ ID NO: 27589 - DNA, 28 bp, synthetic construct
  source 1..28: mol_type = other DNA
ctcctgcctcagcctcccgagtagctgg

SEQ ID NO: 27590 - DNA, 28 bp, synthetic construct
  source 1..28: mol_type = other DNA
tcctgcctcagcctcccgagtagctggg

SEQ ID NO: 27591 - DNA, 28 bp, synthetic construct
  source 1..28: mol_type = other DNA
tcccagctactcgggaggctgaggcagg

SEQ ID NO: 27592 - DNA, 28 bp, synthetic construct
  source 1..28: mol_type = other DNA
gtggtcccagctactcgggaggctgagg

SEQ ID NO: 27593 - DNA, 28 bp, synthetic construct
  source 1..28: mol_type = other DNA
gcatttgtggtcccagctactcgggagg

SEQ ID NO: 27594 - DNA, 28 bp, synthetic construct
  source 1..28: mol_type = other DNA
cgggcatttgtggtcccagctactcggg

SEQ ID NO: 27595 - DNA, 28 bp, synthetic construct
  source 1..28: mol_type = other DNA
gcgggcatttgtggtcccagctactcgg

SEQ ID NO: 27596 - DNA, 28 bp, synthetic construct
  source 1..28: mol_type = other DNA
gaccacaaatgcccgccaccacgcccgg

SEQ ID NO: 27597 - DNA, 28 bp, synthetic construct
  source 1..28: mol_type = other DNA
agccgggcgtggtggcgggcatttgtgg

SEQ ID NO: 27598 - DNA, 28 bp, synthetic construct
  source 1..28: mol_type = other DNA
aaaaaaattagccgggcgtggtggcggg

SEQ ID NO: 27599 - DNA, 28 bp, synthetic construct
  source 1..28: mol_type = other DNA
aaaaaaaattagccgggcgtggtggcgg

SEQ ID NO: 27600 - DNA, 28 bp, synthetic construct
  source 1..28: mol_type = other DNA
acaaaaaaaaattagccgggcgtggtgg

SEQ ID NO: 27601 - DNA, 28 bp, synthetic construct
  source 1..28: mol_type = other DNA
aatacaaaaaaaaattagccgggcgtgg

SEQ ID NO: 27602 - DNA, 28 bp, synthetic construct
  source 1..28: mol_type = other DNA
ctaaaaatacaaaaaaaaattagccggg

SEQ ID NO: 27603 - DNA, 28 bp, synthetic construct
  source 1..28: mol_type = other DNA
actaaaaatacaaaaaaaaattagccgg

SEQ ID NO: 27604 - DNA, 28 bp, synthetic construct
  source 1..28: mol_type = other DNA
tttttttttgtatttttagtagagacgg

SEQ ID NO: 27605 - DNA, 28 bp, synthetic construct
  source 1..28: mol_type = other DNA
ttttttttgtatttttagtagagacggg

SEQ ID NO: 27606 - DNA, 28 bp, synthetic construct
  source 1..28: mol_type = other DNA
tttttttgtatttttagtagagacgggg

SEQ ID NO: 27607 - DNA, 28 bp, synthetic construct
  source 1..28: mol_type = other DNA
gagacggggtttcaccgtgttagccagg

SEQ ID NO: 27608 - DNA, 28 bp, synthetic construct
  source 1..28: mol_type = other DNA
cggggtttcaccgtgttagccaggatgg

SEQ ID NO: 27609 - DNA, 28 bp, synthetic construct
  source 1..28: mol_type = other DNA
gagatcgagaccatcctggctaacacgg

SEQ ID NO: 27610 - DNA, 28 bp, synthetic construct
  source 1..28: mol_type = other DNA
cgaggtcaggagatcgagaccatcctgg

SEQ ID NO: 27611 - DNA, 28 bp, synthetic construct
  source 1..28: mol_type = other DNA
gctgaggcgggcagatcacgaggtcagg

SEQ ID NO: 27612 - DNA, 28 bp, synthetic construct
  source 1..28: mol_type = other DNA
gggaggctgaggcgggcagatcacgagg

SEQ ID NO: 27613 - DNA, 28 bp, synthetic construct
  source 1..28: mol_type = other DNA
tgcccgcctcagcctcccaaagtgctgg

SEQ ID NO: 27614 - DNA, 28 bp, synthetic construct
  source 1..28: mol_type = other DNA
gcccgcctcagcctcccaaagtgctggg

SEQ ID NO: 27615 - DNA, 28 bp, synthetic construct
  source 1..28: mol_type = other DNA
tcccagcactttgggaggctgaggcggg

SEQ ID NO: 27616 - DNA, 28 bp, synthetic construct
  source 1..28: mol_type = other DNA
atcccagcactttgggaggctgaggcgg

SEQ ID NO: 27617 - DNA, 28 bp, synthetic construct
  source 1..28: mol_type = other DNA
gtaatcccagcactttgggaggctgagg

SEQ ID NO: 27618 - DNA, 28 bp, synthetic construct
  source 1..28: mol_type = other DNA
cagcctcccaaagtgctgggattacagg

SEQ ID NO: 27619 - DNA, 28 bp, synthetic construct
  source 1..28: mol_type = other DNA
atgcctgtaatcccagcactttgggagg

SEQ ID NO: 27620 - DNA, 28 bp, synthetic construct
  source 1..28: mol_type = other DNA
cttatgcctgtaatcccagcactttggg

SEQ ID NO: 27621 - DNA, 28 bp, synthetic construct
  source 1..28: mol_type = other DNA
gcttatgcctgtaatcccagcactttgg

SEQ ID NO: 27622 - DNA, 28 bp, synthetic construct
  source 1..28: mol_type = other DNA
gattacaggcataagccaccgcgcctgg

SEQ ID NO: 27623 - DNA, 28 bp, synthetic construct
  source 1..28: mol_type = other DNA
gtaggtatgttcaggccaggcgcggtgg

SEQ ID NO: 27624 - DNA, 28 bp, synthetic construct
  source 1..28: mol_type = other DNA
aaagtaggtatgttcaggccaggcgcgg

SEQ ID NO: 27625 - DNA, 28 bp, synthetic construct
  source 1..28: mol_type = other DNA
cattgaaagtaggtatgttcaggccagg

SEQ ID NO: 27626 - DNA, 28 bp, synthetic construct
  source 1..28: mol_type = other DNA
aaacacattgaaagtaggtatgttcagg

SEQ ID NO: 27627 - DNA, 28 bp, synthetic construct
  source 1..28: mol_type = other DNA
aggagaaagtaaacacattgaaagtagg

SEQ ID NO: 27628 - DNA, 28 bp, synthetic construct
  source 1..28: mol_type = other DNA
tgaaaatattaggaggtgaaataatagg

SEQ ID NO: 27629 - DNA, 28 bp, synthetic construct
  source 1..28: mol_type = other DNA
aatgttattatgtgaaaatattaggagg

SEQ ID NO: 27630 - DNA, 28 bp, synthetic construct
  source 1..28: mol_type = other DNA
ttaaatgttattatgtgaaaatattagg

SEQ ID NO: 27631 - DNA, 28 bp, synthetic construct
  source 1..28: mol_type = other DNA
atatatctcaaagcaaatttcaagaggg

SEQ ID NO: 27632 - DNA, 28 bp, synthetic construct
  source 1..28: mol_type = other DNA
tatatatctcaaagcaaatttcaagagg

SEQ ID NO: 27633 - DNA, 28 bp, synthetic construct
  source 1..28: mol_type = other DNA
aaatttgctttgagatatatatgcatgg

SEQ ID NO: 27634 - DNA, 28 bp, synthetic construct
  source 1..28: mol_type = other DNA
agatatatatgcatggcttaaaataagg

SEQ ID NO: 27635 - DNA, 28 bp, synthetic construct
  source 1..28: mol_type = other DNA
gattctactatagaaataattttgctgg

SEQ ID NO: 27636 - DNA, 28 bp, synthetic construct
  source 1..28: mol_type = other DNA
attctactatagaaataattttgctggg

SEQ ID NO: 27637 - DNA, 28 bp, synthetic construct
  source 1..28: mol_type = other DNA
taattttgctgggttcaaataatgctgg

SEQ ID NO: 27638 - DNA, 28 bp, synthetic construct
  source 1..28: mol_type = other DNA
aattttgctgggttcaaataatgctggg

SEQ ID NO: 27639 - DNA, 28 bp, synthetic construct
  source 1..28: mol_type = other DNA
ttcataagcagtaactgtgcctaaatgg

SEQ ID NO: 27640 - DNA, 28 bp, synthetic construct
  source 1..28: mol_type = other DNA
tgcctaaatggtactgtttaaatacagg

SEQ ID NO: 27641 - DNA, 28 bp, synthetic construct
  source 1..28: mol_type = other DNA
gcctaaatggtactgtttaaatacaggg

SEQ ID NO: 27642 - DNA, 28 bp, synthetic construct
  source 1..28: mol_type = other DNA
tccctgtatttaaacagtaccatttagg

SEQ ID NO: 27643 - DNA, 28 bp, synthetic construct
  source 1..28: mol_type = other DNA
aaatacagggactctcaaaagtctcagg

SEQ ID NO: 27644 - DNA, 28 bp, synthetic construct
  source 1..28: mol_type = other DNA
gatgactttatgtgaagtatacttttgg

SEQ ID NO: 27645 - DNA, 28 bp, synthetic construct
  source 1..28: mol_type = other DNA
ttctgaattctgtgattctcttgaaagg

SEQ ID NO: 27646 - DNA, 28 bp, synthetic construct
  source 1..28: mol_type = other DNA
tttcaagagaatcacagaattcagaagg

SEQ ID NO: 27647 - DNA, 28 bp, synthetic construct
  source 1..28: mol_type = other DNA
cattcatagaatcctcaaactaacttgg

SEQ ID NO: 27648 - DNA, 28 bp, synthetic construct
  source 1..28: mol_type = other DNA
aatcctcaaactaacttggtgttatagg

SEQ ID NO: 27649 - DNA, 28 bp, synthetic construct
  source 1..28: mol_type = other DNA
catcctataacaccaagttagtttgagg

SEQ ID NO: 27650 - DNA, 28 bp, synthetic construct
  source 1..28: mol_type = other DNA
ctcaaactaacttggtgttataggatgg

SEQ ID NO: 27651 - DNA, 28 bp, synthetic construct
  source 1..28: mol_type = other DNA
tataggatggtcttgaaagaaactgagg

SEQ ID NO: 27652 - DNA, 28 bp, synthetic construct
  source 1..28: mol_type = other DNA
gatggtcttgaaagaaactgaggccagg

SEQ ID NO: 27653 - DNA, 28 bp, synthetic construct
  source 1..28: mol_type = other DNA
gattgcaggcatgactcacagcgcctgg

SEQ ID NO: 27654 - DNA, 28 bp, synthetic construct
  source 1..28: mol_type = other DNA
agtcatgcctgcaatcccaatactttgg

SEQ ID NO: 27655 - DNA, 28 bp, synthetic construct
  source 1..28: mol_type = other DNA
gtcatgcctgcaatcccaatactttggg

SEQ ID NO: 27656 - DNA, 28 bp, synthetic construct
  source 1..28: mol_type = other DNA
atgcctgcaatcccaatactttgggagg

SEQ ID NO: 27657 - DNA, 28 bp, synthetic construct
  source 1..28: mol_type = other DNA
cagcctcccaaagtattgggattgcagg

SEQ ID NO: 27658 - DNA, 28 bp, synthetic construct
  source 1..28: mol_type = other DNA
gcaatcccaatactttgggaggctgagg

SEQ ID NO: 27659 - DNA, 28 bp, synthetic construct
  source 1..28: mol_type = other DNA
atcccaatactttgggaggctgaggtgg

SEQ ID NO: 27660 - DNA, 28 bp, synthetic construct
  source 1..28: mol_type = other DNA
tcccaatactttgggaggctgaggtggg

SEQ ID NO: 27661 - DNA, 28 bp, synthetic construct
  source 1..28: mol_type = other DNA
tcccacctcagcctcccaaagtattggg

SEQ ID NO: 27662 - DNA, 28 bp, synthetic construct
  source 1..28: mol_type = other DNA
ctcccacctcagcctcccaaagtattgg

SEQ ID NO: 27663 - DNA, 28 bp, synthetic construct
  source 1..28: mol_type = other DNA
gtgggagaatcacttgagaccagtctgg

SEQ ID NO: 27664 - DNA, 28 bp, synthetic construct
  source 1..28: mol_type = other DNA
tgggagaatcacttgagaccagtctggg

SEQ ID NO: 27665 - DNA, 28 bp, synthetic construct
  source 1..28: mol_type = other DNA
gggggtctgtctgtgttgcccagactgg

SEQ ID NO: 27666 - DNA, 28 bp, synthetic construct
  source 1..28: mol_type = other DNA
ttttaaaattttttaatagagatggggg

SEQ ID NO: 27667 - DNA, 28 bp, synthetic construct
  source 1..28: mol_type = other DNA
attttaaaattttttaatagagatgggg

SEQ ID NO: 27668 - DNA, 28 bp, synthetic construct
  source 1..28: mol_type = other DNA
aattttaaaattttttaatagagatggg

SEQ ID NO: 27669 - DNA, 28 bp, synthetic construct
  source 1..28: mol_type = other DNA
taattttaaaattttttaatagagatgg

SEQ ID NO: 27670 - DNA, 28 bp, synthetic construct
  source 1..28: mol_type = other DNA
ctattaaaaaattttaaaattagcaagg

SEQ ID NO: 27671 - DNA, 28 bp, synthetic construct
  source 1..28: mol_type = other DNA
aaaaaattttaaaattagcaaggcatgg

SEQ ID NO: 27672 - DNA, 28 bp, synthetic construct
  source 1..28: mol_type = other DNA
aaattttaaaattagcaaggcatggtgg

SEQ ID NO: 27673 - DNA, 28 bp, synthetic construct
  source 1..28: mol_type = other DNA
agcaaggcatggtggtacacatctgtgg

SEQ ID NO: 27674 - DNA, 28 bp, synthetic construct
  source 1..28: mol_type = other DNA
gtacacatctgtggtcccagctacttgg

SEQ ID NO: 27675 - DNA, 28 bp, synthetic construct
  source 1..28: mol_type = other DNA
tacacatctgtggtcccagctacttggg

SEQ ID NO: 27676 - DNA, 28 bp, synthetic construct
  source 1..28: mol_type = other DNA
acatctgtggtcccagctacttgggagg

SEQ ID NO: 27677 - DNA, 28 bp, synthetic construct
  source 1..28: mol_type = other DNA
gtcccagctacttgggaggcagaagtgg

SEQ ID NO: 27678 - DNA, 28 bp, synthetic construct
  source 1..28: mol_type = other DNA
tcccagctacttgggaggcagaagtggg

SEQ ID NO: 27679 - DNA, 28 bp, synthetic construct
  source 1..28: mol_type = other DNA
tcccacttctgcctcccaagtagctggg

SEQ ID NO: 27680 - DNA, 28 bp, synthetic construct
  source 1..28: mol_type = other DNA
ctcccacttctgcctcccaagtagctgg

SEQ ID NO: 27681 - DNA, 28 bp, synthetic construct
  source 1..28: mol_type = other DNA
cagctacttgggaggcagaagtgggagg

SEQ ID NO: 27682 - DNA, 28 bp, synthetic construct
  source 1..28: mol_type = other DNA
agaagtgggaggatcacttgagctcagg

SEQ ID NO: 27683 - DNA, 28 bp, synthetic construct
  source 1..28: mol_type = other DNA
agtgggaggatcacttgagctcaggagg

SEQ ID NO: 27684 - DNA, 28 bp, synthetic construct
  source 1..28: mol_type = other DNA
aggctggcatgcagtggcgtgatcacgg

SEQ ID NO: 27685 - DNA, 28 bp, synthetic construct
  source 1..28: mol_type = other DNA
gtgatcacgccactgcatgccagcctgg

SEQ ID NO: 27686 - DNA, 28 bp, synthetic construct
  source 1..28: mol_type = other DNA
ctctgttgtccaggctggcatgcagtgg

SEQ ID NO: 27687 - DNA, 28 bp, synthetic construct
  source 1..28: mol_type = other DNA
cagagtcttgctctgttgtccaggctgg

SEQ ID NO: 27688 - DNA, 28 bp, synthetic construct
  source 1..28: mol_type = other DNA
aagacagagtcttgctctgttgtccagg

SEQ ID NO: 27689 - DNA, 28 bp, synthetic construct
  source 1..28: mol_type = other DNA
tattaaaaaaaaaaaaaaaagagagagg

SEQ ID NO: 27690 - DNA, 28 bp, synthetic construct
  source 1..28: mol_type = other DNA
taaaaaaaaaaaaaaaagagagaggcgg

SEQ ID NO: 27691 - DNA, 28 bp, synthetic construct
  source 1..28: mol_type = other DNA
aaaaaaaaaaaaaaaagagagaggcggg

SEQ ID NO: 27692 - DNA, 28 bp, synthetic construct
  source 1..28: mol_type = other DNA
aaaaaaaaaaaaaaagagagaggcgggg

SEQ ID NO: 27693 - DNA, 28 bp, synthetic construct
  source 1..28: mol_type = other DNA
aaaaaaagagagaggcggggcacagtgg

SEQ ID NO: 27694 - DNA, 28 bp, synthetic construct
  source 1..28: mol_type = other DNA
gctcatgcctgtaatcctagcactttgg

SEQ ID NO: 27695 - DNA, 28 bp, synthetic construct
  source 1..28: mol_type = other DNA
atgcctgtaatcctagcactttggaagg

SEQ ID NO: 27696 - DNA, 28 bp, synthetic construct
  source 1..28: mol_type = other DNA
cagccttccaaagtgctaggattacagg

SEQ ID NO: 27697 - DNA, 28 bp, synthetic construct
  source 1..28: mol_type = other DNA
gtaatcctagcactttggaaggctgagg

SEQ ID NO: 27698 - DNA, 28 bp, synthetic construct
  source 1..28: mol_type = other DNA
atcctagcactttggaaggctgaggtgg

SEQ ID NO: 27699 - DNA, 28 bp, synthetic construct
  source 1..28: mol_type = other DNA
tcctagcactttggaaggctgaggtggg

SEQ ID NO: 27700 - DNA, 28 bp, synthetic construct
  source 1..28: mol_type = other DNA
acccacctcagccttccaaagtgctagg

SEQ ID NO: 27701 - DNA, 28 bp, synthetic construct
  source 1..28: mol_type = other DNA
tagcactttggaaggctgaggtgggtgg

SEQ ID NO: 27702 - DNA, 28 bp, synthetic construct
  source 1..28: mol_type = other DNA
aaggctgaggtgggtggatcgcctgagg

SEQ ID NO: 27703 - DNA, 28 bp, synthetic construct
  source 1..28: mol_type = other DNA
aggctggtctcaaactcttgacctcagg

SEQ ID NO: 27704 - DNA, 28 bp, synthetic construct
  source 1..28: mol_type = other DNA
tgaggtcaagagtttgagaccagcctgg

SEQ ID NO: 27705 - DNA, 28 bp, synthetic construct
  source 1..28: mol_type = other DNA
gagtttgagaccagcctggtcaacacgg

SEQ ID NO: 27706 - DNA, 28 bp, synthetic construct
  source 1..28: mol_type = other DNA
cagggtttcaccgtgttgaccaggctgg

SEQ ID NO: 27707 - DNA, 28 bp, synthetic construct
  source 1..28: mol_type = other DNA
tcagcagggtttcaccgtgttgaccagg

SEQ ID NO: 27708 - DNA, 28 bp, synthetic construct
  source 1..28: mol_type = other DNA
tggtcaacacggtgaaaccctgctgagg

SEQ ID NO: 27709 - DNA, 28 bp, synthetic construct
  source 1..28: mol_type = other DNA
tcaacacggtgaaaccctgctgaggtgg

SEQ ID NO: 27710 - DNA, 28 bp, synthetic construct
  source 1..28: mol_type = other DNA
caacacggtgaaaccctgctgaggtggg

SEQ ID NO: 27711 - DNA, 28 bp, synthetic construct
  source 1..28: mol_type = other DNA
ctcaggcaatctgcccacctcagcaggg

SEQ ID NO: 27712 - DNA, 28 bp, synthetic construct
  source 1..28: mol_type = other DNA
gctcaggcaatctgcccacctcagcagg

SEQ ID NO: 27713 - DNA, 28 bp, synthetic construct
  source 1..28: mol_type = other DNA
tgaggtgggcagattgcctgagctcagg

SEQ ID NO: 27714 - DNA, 28 bp, synthetic construct
  source 1..28: mol_type = other DNA
aggctggtctcaaactcctgagctcagg

SEQ ID NO: 27715 - DNA, 28 bp, synthetic construct
  source 1..28: mol_type = other DNA
tgagctcaggagtttgagaccagcctgg

SEQ ID NO: 27716 - DNA, 28 bp, synthetic construct
  source 1..28: mol_type = other DNA
gagctcaggagtttgagaccagcctggg

SEQ ID NO: 27717 - DNA, 28 bp, synthetic construct
  source 1..28: mol_type = other DNA
gagtttgagaccagcctgggcaacatgg

SEQ ID NO: 27718 - DNA, 28 bp, synthetic construct
  source 1..28: mol_type = other DNA
cagggtttcaccatgttgcccaggctgg

SEQ ID NO: 27719 - DNA, 28 bp, synthetic construct
  source 1..28: mol_type = other DNA
gagacagggtttcaccatgttgcccagg

SEQ ID NO: 27720 - DNA, 28 bp, synthetic construct
  source 1..28: mol_type = other DNA
cactctttttattttagtagagacaggg

SEQ ID NO: 27721 - DNA, 28 bp, synthetic construct
  source 1..28: mol_type = other DNA
tcactctttttattttagtagagacagg

SEQ ID NO: 27722 - DNA, 28 bp, synthetic construct
  source 1..28: mol_type = other DNA
ctctactaaaataaaaagagtgagctgg

SEQ ID NO: 27723 - DNA, 28 bp, synthetic construct
  source 1..28: mol_type = other DNA
tctactaaaataaaaagagtgagctggg

SEQ ID NO: 27724 - DNA, 28 bp, synthetic construct
  source 1..28: mol_type = other DNA
agtgagctgggcaaaaagagtgagctgg

SEQ ID NO: 27725 - DNA, 28 bp, synthetic construct
  source 1..28: mol_type = other DNA
gtgagctgggcaaaaagagtgagctggg

SEQ ID NO: 27726 - DNA, 28 bp, synthetic construct
  source 1..28: mol_type = other DNA
ggcaaaaagagtgagctgggcgtcatgg

SEQ ID NO: 27727 - DNA, 28 bp, synthetic construct
  source 1..28: mol_type = other DNA
gcatgtgtctgtagtcccagctactcgg

SEQ ID NO: 27728 - DNA, 28 bp, synthetic construct
  source 1..28: mol_type = other DNA
gtgtctgtagtcccagctactcggaagg

SEQ ID NO: 27729 - DNA, 28 bp, synthetic construct
  source 1..28: mol_type = other DNA
gtagtcccagctactcggaaggctgagg

SEQ ID NO: 27730 - DNA, 28 bp, synthetic construct
  source 1..28: mol_type = other DNA
tcgttcctcagccttccgagtagctggg

SEQ ID NO: 27731 - DNA, 28 bp, synthetic construct
  source 1..28: mol_type = other DNA
ctcgttcctcagccttccgagtagctgg

SEQ ID NO: 27732 - DNA, 28 bp, synthetic construct
  source 1..28: mol_type = other DNA
tgaggaacgagaattgcttgaacccagg

SEQ ID NO: 27733 - DNA, 28 bp, synthetic construct
  source 1..28: mol_type = other DNA
ggaacgagaattgcttgaacccaggagg

SEQ ID NO: 27734 - DNA, 28 bp, synthetic construct
  source 1..28: mol_type = other DNA
acgagaattgcttgaacccaggaggcgg

SEQ ID NO: 27735 - DNA, 28 bp, synthetic construct
  source 1..28: mol_type = other DNA
agaattgcttgaacccaggaggcggagg

SEQ ID NO: 27736 - DNA, 28 bp, synthetic construct
  source 1..28: mol_type = other DNA
cggctcactgcaacctccgcctcctggg

SEQ ID NO: 27737 - DNA, 28 bp, synthetic construct
  source 1..28: mol_type = other DNA
tcggctcactgcaacctccgcctcctgg

SEQ ID NO: 27738 - DNA, 28 bp, synthetic construct
  source 1..28: mol_type = other DNA
gggctggagtgcagtggcgttatctcgg

SEQ ID NO: 27739 - DNA, 28 bp, synthetic construct
  source 1..28: mol_type = other DNA
ggagtggggtggggctggagtgcagtgg

SEQ ID NO: 27740 - DNA, 28 bp, synthetic construct
  source 1..28: mol_type = other DNA
tttttttttgggagtggggtggggctgg

SEQ ID NO: 27741 - DNA, 28 bp, synthetic construct
  source 1..28: mol_type = other DNA
tggttttttttttgggagtggggtgggg

SEQ ID NO: 27742 - DNA, 28 bp, synthetic construct
  source 1..28: mol_type = other DNA
ttggttttttttttgggagtggggtggg

SEQ ID NO: 27743 - DNA, 28 bp, synthetic construct
  source 1..28: mol_type = other DNA
tttggttttttttttgggagtggggtgg

SEQ ID NO: 27744 - DNA, 28 bp, synthetic construct
  source 1..28: mol_type = other DNA
ttttttggttttttttttgggagtgggg

SEQ ID NO: 27745 - DNA, 28 bp, synthetic construct
  source 1..28: mol_type = other DNA
gttttttggttttttttttgggagtggg

SEQ ID NO: 27746 - DNA, 28 bp, synthetic construct
  source 1..28: mol_type = other DNA
tgttttttggttttttttttgggagtgg

SEQ ID NO: 27747 - DNA, 28 bp, synthetic construct
  source 1..28: mol_type = other DNA
ttttttgttttttggttttttttttggg

SEQ ID NO: 27748 - DNA, 28 bp, synthetic construct
  source 1..28: mol_type = other DNA
gttttttgttttttggttttttttttgg

SEQ ID NO: 27749 - DNA, 28 bp, synthetic construct
  source 1..28: mol_type = other DNA
aaaaaaccaaaaaacaaaaaactaaagg

SEQ ID NO: 27750 - DNA, 28 bp, synthetic construct
  source 1..28: mol_type = other DNA
ttttaacctttagttttttgttttttgg

SEQ ID NO: 27751 - DNA, 28 bp, synthetic construct
  source 1..28: mol_type = other DNA
ttgttcagcatttgtttttctaaagtgg

SEQ ID NO: 27752 - DNA, 28 bp, synthetic construct
  source 1..28: mol_type = other DNA
catatgaactagctattctactccaagg

SEQ ID NO: 27753 - DNA, 28 bp, synthetic construct
  source 1..28: mol_type = other DNA
attcgtttctcttgggtatgtgccttgg

SEQ ID NO: 27754 - DNA, 28 bp, synthetic construct
  source 1..28: mol_type = other DNA
gtgaatgtatgtattcgtttctcttggg

SEQ ID NO: 27755 - DNA, 28 bp, synthetic construct
  source 1..28: mol_type = other DNA
tgtgaatgtatgtattcgtttctcttgg

SEQ ID NO: 27756 - DNA, 28 bp, synthetic construct
  source 1..28: mol_type = other DNA
gaatacatacattcacacaaaaacttgg

SEQ ID NO: 27757 - DNA, 28 bp, synthetic construct
  source 1..28: mol_type = other DNA
acaaaaacttggacacatatgttcatgg

SEQ ID NO: 27758 - DNA, 28 bp, synthetic construct
  source 1..28: mol_type = other DNA
ctaaaacaatcatttgtccatcaactgg

SEQ ID NO: 27759 - DNA, 28 bp, synthetic construct
  source 1..28: mol_type = other DNA
aatcatttgtccatcaactggtgaatgg

SEQ ID NO: 27760 - DNA, 28 bp, synthetic construct
  source 1..28: mol_type = other DNA
ttttgtttatccattcaccagttgatgg

SEQ ID NO: 27761 - DNA, 28 bp, synthetic construct
  source 1..28: mol_type = other DNA
tcaactggtgaatggataaacaaaatgg

SEQ ID NO: 27762 - DNA, 28 bp, synthetic construct
  source 1..28: mol_type = other DNA
aacaaaatggtatatatctatataatgg

SEQ ID NO: 27763 - DNA, 28 bp, synthetic construct
  source 1..28: mol_type = other DNA
attatgctaagttaaagaaaccagccgg

SEQ ID NO: 27764 - DNA, 28 bp, synthetic construct
  source 1..28: mol_type = other DNA
ttatgctaagttaaagaaaccagccggg

SEQ ID NO: 27765 - DNA, 28 bp, synthetic construct
  source 1..28: mol_type = other DNA
ctaagttaaagaaaccagccgggcgcgg

SEQ ID NO: 27766 - DNA, 28 bp, synthetic construct
  source 1..28: mol_type = other DNA
agttaaagaaaccagccgggcgcggtgg

SEQ ID NO: 27767 - DNA, 28 bp, synthetic construct
  source 1..28: mol_type = other DNA
acaggcgtgagccaccgcgcccggctgg

SEQ ID NO: 27768 - DNA, 28 bp, synthetic construct
  source 1..28: mol_type = other DNA
ggttacaggcgtgagccaccgcgcccgg

SEQ ID NO: 27769 - DNA, 28 bp, synthetic construct
  source 1..28: mol_type = other DNA
gctcacgcctgtaaccctagcactttgg

SEQ ID NO: 27770 - DNA, 28 bp, synthetic construct
  source 1..28: mol_type = other DNA
ctcacgcctgtaaccctagcactttggg

SEQ ID NO: 27771 - DNA, 28 bp, synthetic construct
  source 1..28: mol_type = other DNA
acgcctgtaaccctagcactttgggagg

SEQ ID NO: 27772 - DNA, 28 bp, synthetic construct
  source 1..28: mol_type = other DNA
cggcctcccaaagtgctagggttacagg

SEQ ID NO: 27773 - DNA, 28 bp, synthetic construct
  source 1..28: mol_type = other DNA
gtaaccctagcactttgggaggccgagg

SEQ ID NO: 27774 - DNA, 28 bp, synthetic construct
  source 1..28: mol_type = other DNA
ccctagcactttgggaggccgaggcagg

SEQ ID NO: 27775 - DNA, 28 bp, synthetic construct
  source 1..28: mol_type = other DNA
acctgcctcggcctcccaaagtgctagg

SEQ ID NO: 27776 - DNA, 28 bp, synthetic construct
  source 1..28: mol_type = other DNA
tagcactttgggaggccgaggcaggtgg

SEQ ID NO: 27777 - DNA, 28 bp, synthetic construct
  source 1..28: mol_type = other DNA
gggaggccgaggcaggtggatcacgagg

SEQ ID NO: 27778 - DNA, 28 bp, synthetic construct
  source 1..28: mol_type = other DNA
gccgaggcaggtggatcacgaggtcagg

SEQ ID NO: 27779 - DNA, 28 bp, synthetic construct
  source 1..28: mol_type = other DNA
tcctgacctcgtgatccacctgcctcgg

SEQ ID NO: 27780 - DNA, 28 bp, synthetic construct
  source 1..28: mol_type = other DNA
cgaggtcaggagatcgagaccatcctgg

SEQ ID NO: 27781 - DNA, 28 bp, synthetic construct
  source 1..28: mol_type = other DNA
tggggtttcactgtgttagccaggatgg

SEQ ID NO: 27782 - DNA, 28 bp, synthetic construct
  source 1..28: mol_type = other DNA
gagatggggtttcactgtgttagccagg

SEQ ID NO: 27783 - DNA, 28 bp, synthetic construct
  source 1..28: mol_type = other DNA
attttttgtatttttagtagagatgggg

SEQ ID NO: 27784 - DNA, 28 bp, synthetic construct
  source 1..28: mol_type = other DNA
aattttttgtatttttagtagagatggg

SEQ ID NO: 27785 - DNA, 28 bp, synthetic construct
  source 1..28: mol_type = other DNA
taattttttgtatttttagtagagatgg

SEQ ID NO: 27786 - DNA, 28 bp, synthetic construct
  source 1..28: mol_type = other DNA
tctactaaaaatacaaaaaattagccgg

SEQ ID NO: 27787 - DNA, 28 bp, synthetic construct
  source 1..28: mol_type = other DNA
ctactaaaaatacaaaaaattagccggg

SEQ ID NO: 27788 - DNA, 28 bp, synthetic construct
  source 1..28: mol_type = other DNA
aaaaatacaaaaaattagccgggtgtgg

SEQ ID NO: 27789 - DNA, 28 bp, synthetic construct
  source 1..28: mol_type = other DNA
aatacaaaaaattagccgggtgtggtgg

SEQ ID NO: 27790 - DNA, 28 bp, synthetic construct
  source 1..28: mol_type = other DNA
acaaaaaattagccgggtgtggtggcgg

SEQ ID NO: 27791 - DNA, 28 bp, synthetic construct
  source 1..28: mol_type = other DNA
caaaaaattagccgggtgtggtggcggg

SEQ ID NO: 27792 - DNA, 28 bp, synthetic construct
  source 1..28: mol_type = other DNA
gactacaggcgcccgccaccacacccgg

SEQ ID NO: 27793 - DNA, 28 bp, synthetic construct
  source 1..28: mol_type = other DNA
ggcgggcgcctgtagtcccagctactgg

SEQ ID NO: 27794 - DNA, 28 bp, synthetic construct
  source 1..28: mol_type = other DNA
gcgggcgcctgtagtcccagctactggg

SEQ ID NO: 27795 - DNA, 28 bp, synthetic construct
  source 1..28: mol_type = other DNA
cgggcgcctgtagtcccagctactgggg

SEQ ID NO: 27796 - DNA, 28 bp, synthetic construct
  source 1..28: mol_type = other DNA
gcgcctgtagtcccagctactggggagg

SEQ ID NO: 27797 - DNA, 28 bp, synthetic construct
  source 1..28: mol_type = other DNA
cagcctccccagtagctgggactacagg

SEQ ID NO: 27798 - DNA, 28 bp, synthetic construct
  source 1..28: mol_type = other DNA
gtagtcccagctactggggaggctgagg

SEQ ID NO: 27799 - DNA, 28 bp, synthetic construct
  source 1..28: mol_type = other DNA
tcccagctactggggaggctgaggcagg

SEQ ID NO: 27800 - DNA, 28 bp, synthetic construct
  source 1..28: mol_type = other DNA
tcctgcctcagcctccccagtagctggg

SEQ ID NO: 27801 - DNA, 28 bp, synthetic construct
  source 1..28: mol_type = other DNA
ctcctgcctcagcctccccagtagctgg

SEQ ID NO: 27802 - DNA, 28 bp, synthetic construct
  source 1..28: mol_type = other DNA
tactggggaggctgaggcaggagaatgg

SEQ ID NO: 27803 - DNA, 28 bp, synthetic construct
  source 1..28: mol_type = other DNA
tgaggcaggagaatggcgtgaacccagg

SEQ ID NO: 27804 - DNA, 28 bp, synthetic construct
  source 1..28: mol_type = other DNA
ggcaggagaatggcgtgaacccaggagg

SEQ ID NO: 27805 - DNA, 28 bp, synthetic construct
  source 1..28: mol_type = other DNA
aggagaatggcgtgaacccaggaggcgg

SEQ ID NO: 27806 - DNA, 28 bp, synthetic construct
  source 1..28: mol_type = other DNA
ggagaatggcgtgaacccaggaggcggg

SEQ ID NO: 27807 - DNA, 28 bp, synthetic construct
  source 1..28: mol_type = other DNA
gagaatggcgtgaacccaggaggcgggg

SEQ ID NO: 27808 - DNA, 28 bp, synthetic construct
  source 1..28: mol_type = other DNA
tggctcactgcaagccccgcctcctggg

SEQ ID NO: 27809 - DNA, 28 bp, synthetic construct
  source 1..28: mol_type = other DNA
ttggctcactgcaagccccgcctcctgg

SEQ ID NO: 27810 - DNA, 28 bp, synthetic construct
  source 1..28: mol_type = other DNA
aggctggagtgcagtggtgcaatcttgg

SEQ ID NO: 27811 - DNA, 28 bp, synthetic construct
  source 1..28: mol_type = other DNA
agattgcaccactgcactccagcctagg

SEQ ID NO: 27812 - DNA, 28 bp, synthetic construct
  source 1..28: mol_type = other DNA
ctctgtcgcctaggctggagtgcagtgg

SEQ ID NO: 27813 - DNA, 28 bp, synthetic construct
  source 1..28: mol_type = other DNA
aggagtctggctctgtcgcctaggctgg

SEQ ID NO: 27814 - DNA, 28 bp, synthetic construct
  source 1..28: mol_type = other DNA
tgagaggagtctggctctgtcgcctagg

SEQ ID NO: 27815 - DNA, 28 bp, synthetic construct
  source 1..28: mol_type = other DNA
ttttgttttgtttttgagaggagtctgg

SEQ ID NO: 27816 - DNA, 28 bp, synthetic construct
  source 1..28: mol_type = other DNA
tgttttgttttgttttgtttttgagagg

SEQ ID NO: 27817 - DNA, 28 bp, synthetic construct
  source 1..28: mol_type = other DNA
aaaaacagatacaaaagactacacatgg

SEQ ID NO: 27818 - DNA, 28 bp, synthetic construct
  source 1..28: mol_type = other DNA
aaaagactacacatggtatgagaccagg

SEQ ID NO: 27819 - DNA, 28 bp, synthetic construct
  source 1..28: mol_type = other DNA
actacacatggtatgagaccaggacagg

SEQ ID NO: 27820 - DNA, 28 bp, synthetic construct
  source 1..28: mol_type = other DNA
ctacacatggtatgagaccaggacaggg

SEQ ID NO: 27821 - DNA, 28 bp, synthetic construct
  source 1..28: mol_type = other DNA
ggtatgagaccaggacagggaaatctgg

SEQ ID NO: 27822 - DNA, 28 bp, synthetic construct
  source 1..28: mol_type = other DNA
tttctgtctccagatttccctgtcctgg

SEQ ID NO: 27823 - DNA, 28 bp, synthetic construct
  source 1..28: mol_type = other DNA
aatctggagacagaaagtagattagtgg

SEQ ID NO: 27824 - DNA, 28 bp, synthetic construct
  source 1..28: mol_type = other DNA
gacagaaagtagattagtggttgtcagg

SEQ ID NO: 27825 - DNA, 28 bp, synthetic construct
  source 1..28: mol_type = other DNA
acagaaagtagattagtggttgtcaggg

SEQ ID NO: 27826 - DNA, 28 bp, synthetic construct
  source 1..28: mol_type = other DNA
cagaaagtagattagtggttgtcagggg

SEQ ID NO: 27827 - DNA, 28 bp, synthetic construct
  source 1..28: mol_type = other DNA
aagtagattagtggttgtcaggggttgg

SEQ ID NO: 27828 - DNA, 28 bp, synthetic construct
  source 1..28: mol_type = other DNA
agtagattagtggttgtcaggggttggg

SEQ ID NO: 27829 - DNA, 28 bp, synthetic construct
  source 1..28: mol_type = other DNA
ttagtggttgtcaggggttgggatgtgg

SEQ ID NO: 27830 - DNA, 28 bp, synthetic construct
  source 1..28: mol_type = other DNA
tagtggttgtcaggggttgggatgtggg

SEQ ID NO: 27831 - DNA, 28 bp, synthetic construct
  source 1..28: mol_type = other DNA
tcaggggttgggatgtgggtgagaatgg

SEQ ID NO: 27832 - DNA, 28 bp, synthetic construct
  source 1..28: mol_type = other DNA
taactgtatgtacccagtctctccttgg

SEQ ID NO: 27833 - DNA, 28 bp, synthetic construct
  source 1..28: mol_type = other DNA
aactgtatgtacccagtctctccttggg

SEQ ID NO: 27834 - DNA, 28 bp, synthetic construct
  source 1..28: mol_type = other DNA
actgtatgtacccagtctctccttgggg

SEQ ID NO: 27835 - DNA, 28 bp, synthetic construct
  source 1..28: mol_type = other DNA
attttcaacaccccaaggagagactggg

SEQ ID NO: 27836 - DNA, 28 bp, synthetic construct
  source 1..28: mol_type = other DNA
tattttcaacaccccaaggagagactgg

SEQ ID NO: 27837 - DNA, 28 bp, synthetic construct
  source 1..28: mol_type = other DNA
atttcagaatattttcaacaccccaagg

SEQ ID NO: 27838 - DNA, 28 bp, synthetic construct
  source 1..28: mol_type = other DNA
gtggtttttagtatattcacagctgtgg

SEQ ID NO: 27839 - DNA, 28 bp, synthetic construct
  source 1..28: mol_type = other DNA
taaaaaccactaaactgtaccttttagg

SEQ ID NO: 27840 - DNA, 28 bp, synthetic construct
  source 1..28: mol_type = other DNA
aattcacctaaaaggtacagtttagtgg

SEQ ID NO: 27841 - DNA, 28 bp, synthetic construct
  source 1..28: mol_type = other DNA
aactgtaccttttaggtgaattttatgg

SEQ ID NO: 27842 - DNA, 28 bp, synthetic construct
  source 1..28: mol_type = other DNA
tcacataccataaaattcacctaaaagg

SEQ ID NO: 27843 - DNA, 28 bp, synthetic construct
  source 1..28: mol_type = other DNA
attttatggtatgtgaaatatatctcgg

SEQ ID NO: 27844 - DNA, 28 bp, synthetic construct
  source 1..28: mol_type = other DNA
tatggtatgtgaaatatatctcggccgg

SEQ ID NO: 27845 - DNA, 28 bp, synthetic construct
  source 1..28: mol_type = other DNA
atggtatgtgaaatatatctcggccggg

SEQ ID NO: 27846 - DNA, 28 bp, synthetic construct
  source 1..28: mol_type = other DNA
atgtgaaatatatctcggccgggcgtgg

SEQ ID NO: 27847 - DNA, 28 bp, synthetic construct
  source 1..28: mol_type = other DNA
tgaaatatatctcggccgggcgtggtgg

SEQ ID NO: 27848 - DNA, 28 bp, synthetic construct
  source 1..28: mol_type = other DNA
gattacaggcatgagccaccacgcccgg

SEQ ID NO: 27849 - DNA, 28 bp, synthetic construct
  source 1..28: mol_type = other DNA
gctcatgcctgtaatcccagcactttgg

SEQ ID NO: 27850 - DNA, 28 bp, synthetic construct
  source 1..28: mol_type = other DNA
ctcatgcctgtaatcccagcactttggg

SEQ ID NO: 27851 - DNA, 28 bp, synthetic construct
  source 1..28: mol_type = other DNA
atgcctgtaatcccagcactttgggagg

SEQ ID NO: 27852 - DNA, 28 bp, synthetic construct
  source 1..28: mol_type = other DNA
cggcctcccaaagtgctgggattacagg

SEQ ID NO: 27853 - DNA, 28 bp, synthetic construct
  source 1..28: mol_type = other DNA
gtaatcccagcactttgggaggccgagg

SEQ ID NO: 27854 - DNA, 28 bp, synthetic construct
  source 1..28: mol_type = other DNA
atttgcctcggcctcccaaagtgctggg

SEQ ID NO: 27855 - DNA, 28 bp, synthetic construct
  source 1..28: mol_type = other DNA
gatttgcctcggcctcccaaagtgctgg

SEQ ID NO: 27856 - DNA, 28 bp, synthetic construct
  source 1..28: mol_type = other DNA
ctttgggaggccgaggcaaatcacgagg

SEQ ID NO: 27857 - DNA, 28 bp, synthetic construct
  source 1..28: mol_type = other DNA
ggaggccgaggcaaatcacgaggtcagg

SEQ ID NO: 27858 - DNA, 28 bp, synthetic construct
  source 1..28: mol_type = other DNA
gatctcctgacctcgtgatttgcctcgg

SEQ ID NO: 27859 - DNA, 28 bp, synthetic construct
  source 1..28: mol_type = other DNA
cgaggtcaggagatcgagaccatcctgg

SEQ ID NO: 27860 - DNA, 28 bp, synthetic construct
  source 1..28: mol_type = other DNA
gagatcgagaccatcctggctaacatgg

SEQ ID NO: 27861 - DNA, 28 bp, synthetic construct
  source 1..28: mol_type = other DNA
tggagtttcaccatgttagccaggatgg

SEQ ID NO: 27862 - DNA, 28 bp, synthetic construct
  source 1..28: mol_type = other DNA
gagatggagtttcaccatgttagccagg

SEQ ID NO: 27863 - DNA, 28 bp, synthetic construct
  source 1..28: mol_type = other DNA
aattttttgtattttttagtagagatgg

SEQ ID NO: 27864 - DNA, 28 bp, synthetic construct
  source 1..28: mol_type = other DNA
ctactaaaaaatacaaaaaattagctgg

SEQ ID NO: 27865 - DNA, 28 bp, synthetic construct
  source 1..28: mol_type = other DNA
aaaaatacaaaaaattagctggccatgg

SEQ ID NO: 27866 - DNA, 28 bp, synthetic construct
  source 1..28: mol_type = other DNA
aatacaaaaaattagctggccatggtgg

SEQ ID NO: 27867 - DNA, 28 bp, synthetic construct
  source 1..28: mol_type = other DNA
acaaaaaattagctggccatggtggtgg

SEQ ID NO: 27868 - DNA, 28 bp, synthetic construct
  source 1..28: mol_type = other DNA
caaaaaattagctggccatggtggtggg

SEQ ID NO: 27869 - DNA, 28 bp, synthetic construct
  source 1..28: mol_type = other DNA
ctgggactacaggtgcccaccaccatgg

SEQ ID NO: 27870 - DNA, 28 bp, synthetic construct
  source 1..28: mol_type = other DNA
gtgggcacctgtagtcccagctactcgg

SEQ ID NO: 27871 - DNA, 28 bp, synthetic construct
  source 1..28: mol_type = other DNA
tgggcacctgtagtcccagctactcggg

SEQ ID NO: 27872 - DNA, 28 bp, synthetic construct
  source 1..28: mol_type = other DNA
cagtgtcccgagtagctgggactacagg

SEQ ID NO: 27873 - DNA, 28 bp, synthetic construct
  source 1..28: mol_type = other DNA
gtagtcccagctactcgggacactgagg

SEQ ID NO: 27874 - DNA, 28 bp, synthetic construct
  source 1..28: mol_type = other DNA
tcccagctactcgggacactgaggcagg

SEQ ID NO: 27875 - DNA, 28 bp, synthetic construct
  source 1..28: mol_type = other DNA
tcctgcctcagtgtcccgagtagctggg

SEQ ID NO: 27876 - DNA, 28 bp, synthetic construct
  source 1..28: mol_type = other DNA
ctcctgcctcagtgtcccgagtagctgg

SEQ ID NO: 27877 - DNA, 28 bp, synthetic construct
  source 1..28: mol_type = other DNA
ggcaggagaattgcttgaacccagaagg

SEQ ID NO: 27878 - DNA, 28 bp, synthetic construct
  source 1..28: mol_type = other DNA
aggagaattgcttgaacccagaaggcgg

SEQ ID NO: 27879 - DNA, 28 bp, synthetic construct
  source 1..28: mol_type = other DNA
agaattgcttgaacccagaaggcggtgg

SEQ ID NO: 27880 - DNA, 28 bp, synthetic construct
  source 1..28: mol_type = other DNA
cggctcactgcaaccaccgccttctggg

SEQ ID NO: 27881 - DNA, 28 bp, synthetic construct
  source 1..28: mol_type = other DNA
tcggctcactgcaaccaccgccttctgg

SEQ ID NO: 27882 - DNA, 28 bp, synthetic construct
  source 1..28: mol_type = other DNA
tggaatgcagtgagtggcgcgatctcgg

SEQ ID NO: 27883 - DNA, 28 bp, synthetic construct
  source 1..28: mol_type = other DNA
agcctctcgctcggggcggaagtggcgg

SEQ ID NO: 27884 - DNA, 28 bp, synthetic construct
  source 1..28: mol_type = other DNA
tctagcctctcgctcggggcggaagtgg

SEQ ID NO: 27885 - DNA, 28 bp, synthetic construct
  source 1..28: mol_type = other DNA
acttccgccccgagcgagaggctagagg

SEQ ID NO: 27886 - DNA, 28 bp, synthetic construct
  source 1..28: mol_type = other DNA
ctcgcctctagcctctcgctcggggcgg

SEQ ID NO: 27887 - DNA, 28 bp, synthetic construct
  source 1..28: mol_type = other DNA
cctctcgcctctagcctctcgctcgggg

SEQ ID NO: 27888 - DNA, 28 bp, synthetic construct
  source 1..28: mol_type = other DNA
gcctctcgcctctagcctctcgctcggg

SEQ ID NO: 27889 - DNA, 28 bp, synthetic construct
  source 1..28: mol_type = other DNA
cgcctctcgcctctagcctctcgctcgg

SEQ ID NO: 27890 - DNA, 28 bp, synthetic construct
  source 1..28: mol_type = other DNA
cgagcgagaggctagaggcgagaggcgg

SEQ ID NO: 27891 - DNA, 28 bp, synthetic construct
  source 1..28: mol_type = other DNA
gagcgagaggctagaggcgagaggcggg

SEQ ID NO: 27892 - DNA, 28 bp, synthetic construct
  source 1..28: mol_type = other DNA
agcgagaggctagaggcgagaggcgggg

SEQ ID NO: 27893 - DNA, 28 bp, synthetic construct
  source 1..28: mol_type = other DNA
gcgagaggctagaggcgagaggcggggg

SEQ ID NO: 27894 - DNA, 28 bp, synthetic construct
  source 1..28: mol_type = other DNA
agaggctagaggcgagaggcgggggagg

SEQ ID NO: 27895 - DNA, 28 bp, synthetic construct
  source 1..28: mol_type = other DNA
ggctagaggcgagaggcgggggaggcgg

SEQ ID NO: 27896 - DNA, 28 bp, synthetic construct
  source 1..28: mol_type = other DNA
gctagaggcgagaggcgggggaggcggg

SEQ ID NO: 27897 - DNA, 28 bp, synthetic construct
  source 1..28: mol_type = other DNA
agaggcgagaggcgggggaggcgggagg

SEQ ID NO: 27898 - DNA, 28 bp, synthetic construct
  source 1..28: mol_type = other DNA
gaggcgagaggcgggggaggcgggaggg

SEQ ID NO: 27899 - DNA, 28 bp, synthetic construct
  source 1..28: mol_type = other DNA
ggcgggggaggcgggagggaccctgcgg

SEQ ID NO: 27900 - DNA, 28 bp, synthetic construct
  source 1..28: mol_type = other DNA
gggaggcgggagggaccctgcggacagg

SEQ ID NO: 27901 - DNA, 28 bp, synthetic construct
  source 1..28: mol_type = other DNA
ggaggcgggagggaccctgcggacaggg

SEQ ID NO: 27902 - DNA, 28 bp, synthetic construct
  source 1..28: mol_type = other DNA
ggaccctgcggacagggcacgagtccgg

SEQ ID NO: 27903 - DNA, 28 bp, synthetic construct
  source 1..28: mol_type = other DNA
gaccctgcggacagggcacgagtccggg

SEQ ID NO: 27904 - DNA, 28 bp, synthetic construct
  source 1..28: mol_type = other DNA
gacccggactcgtgccctgtccgcaggg

SEQ ID NO: 27905 - DNA, 28 bp, synthetic construct
  source 1..28: mol_type = other DNA
agacccggactcgtgccctgtccgcagg

SEQ ID NO: 27906 - DNA, 28 bp, synthetic construct
  source 1..28: mol_type = other DNA
gcggacagggcacgagtccgggtctcgg

SEQ ID NO: 27907 - DNA, 28 bp, synthetic construct
  source 1..28: mol_type = other DNA
gacagggcacgagtccgggtctcggagg

SEQ ID NO: 27908 - DNA, 28 bp, synthetic construct
  source 1..28: mol_type = other DNA
agggcacgagtccgggtctcggaggagg

SEQ ID NO: 27909 - DNA, 28 bp, synthetic construct
  source 1..28: mol_type = other DNA
cacgagtccgggtctcggaggaggtcgg

SEQ ID NO: 27910 - DNA, 28 bp, synthetic construct
  source 1..28: mol_type = other DNA
gcagtcgccgacctcctccgagacccgg

SEQ ID NO: 27911 - DNA, 28 bp, synthetic construct
  source 1..28: mol_type = other DNA
tcggaggaggtcggcgactgccgcgtgg

SEQ ID NO: 27912 - DNA, 28 bp, synthetic construct
  source 1..28: mol_type = other DNA
cggaggaggtcggcgactgccgcgtggg

SEQ ID NO: 27913 - DNA, 28 bp, synthetic construct
  source 1..28: mol_type = other DNA
gagctggcgcgagcagagcctgcgccgg

SEQ ID NO: 27914 - DNA, 28 bp, synthetic construct
  source 1..28: mol_type = other DNA
ctggcgcgagcagagcctgcgccggcgg

SEQ ID NO: 27915 - DNA, 28 bp, synthetic construct
  source 1..28: mol_type = other DNA
gcgagcagagcctgcgccggcggagagg

SEQ ID NO: 27916 - DNA, 28 bp, synthetic construct
  source 1..28: mol_type = other DNA
agagcctgcgccggcggagaggctcagg

SEQ ID NO: 27917 - DNA, 28 bp, synthetic construct
  source 1..28: mol_type = other DNA
ggggcctgagcctctccgccggcgcagg

SEQ ID NO: 27918 - DNA, 28 bp, synthetic construct
  source 1..28: mol_type = other DNA
tcgtgcggggcctgagcctctccgccgg

SEQ ID NO: 27919 - DNA, 28 bp, synthetic construct
  source 1..28: mol_type = other DNA
ggagaggctcaggccccgcacgatccgg

SEQ ID NO: 27920 - DNA, 28 bp, synthetic construct
  source 1..28: mol_type = other DNA
gagaggctcaggccccgcacgatccggg

SEQ ID NO: 27921 - DNA, 28 bp, synthetic construct
  source 1..28: mol_type = other DNA
agaggctcaggccccgcacgatccgggg

SEQ ID NO: 27922 - DNA, 28 bp, synthetic construct
  source 1..28: mol_type = other DNA
gccccgcacgatccggggagagcgctgg

SEQ ID NO: 27923 - DNA, 28 bp, synthetic construct
  source 1..28: mol_type = other DNA
gccagcgctctccccggatcgtgcgggg

SEQ ID NO: 27924 - DNA, 28 bp, synthetic construct
  source 1..28: mol_type = other DNA
cgccagcgctctccccggatcgtgcggg

SEQ ID NO: 27925 - DNA, 28 bp, synthetic construct
  source 1..28: mol_type = other DNA
gcgccagcgctctccccggatcgtgcgg

SEQ ID NO: 27926 - DNA, 28 bp, synthetic construct
  source 1..28: mol_type = other DNA
cgatccggggagagcgctggcgctgcgg

SEQ ID NO: 27927 - DNA, 28 bp, synthetic construct
  source 1..28: mol_type = other DNA
tgcgccgcagcgccagcgctctccccgg

SEQ ID NO: 27928 - DNA, 28 bp, synthetic construct
  source 1..28: mol_type = other DNA
cagggcttggcgtgggggcggggcgcgg

SEQ ID NO: 27929 - DNA, 28 bp, synthetic construct
  source 1..28: mol_type = other DNA
gccccgcccccacgccaagccctgtcgg

SEQ ID NO: 27930 - DNA, 28 bp, synthetic construct
  source 1..28: mol_type = other DNA
gccgacagggcttggcgtgggggcgggg

SEQ ID NO: 27931 - DNA, 28 bp, synthetic construct
  source 1..28: mol_type = other DNA
ggccgacagggcttggcgtgggggcggg

SEQ ID NO: 27932 - DNA, 28 bp, synthetic construct
  source 1..28: mol_type = other DNA
cggccgacagggcttggcgtgggggcgg

SEQ ID NO: 27933 - DNA, 28 bp, synthetic construct
  source 1..28: mol_type = other DNA
cccccacgccaagccctgtcggccgtgg

SEQ ID NO: 27934 - DNA, 28 bp, synthetic construct
  source 1..28: mol_type = other DNA
cccacggccgacagggcttggcgtgggg

SEQ ID NO: 27935 - DNA, 28 bp, synthetic construct
  source 1..28: mol_type = other DNA
ccccacggccgacagggcttggcgtggg

SEQ ID NO: 27936 - DNA, 28 bp, synthetic construct
  source 1..28: mol_type = other DNA
tccccacggccgacagggcttggcgtgg

SEQ ID NO: 27937 - DNA, 28 bp, synthetic construct
  source 1..28: mol_type = other DNA
tactttccccacggccgacagggcttgg

SEQ ID NO: 27938 - DNA, 28 bp, synthetic construct
  source 1..28: mol_type = other DNA
ccaggtactttccccacggccgacaggg

SEQ ID NO: 27939 - DNA, 28 bp, synthetic construct
  source 1..28: mol_type = other DNA
tccaggtactttccccacggccgacagg

SEQ ID NO: 27940 - DNA, 28 bp, synthetic construct
  source 1..28: mol_type = other DNA
gccgtggggaaagtacctggagcgtcgg

SEQ ID NO: 27941 - DNA, 28 bp, synthetic construct
  source 1..28: mol_type = other DNA
tccgacgctccaggtactttccccacgg

SEQ ID NO: 27942 - DNA, 28 bp, synthetic construct
  source 1..28: mol_type = other DNA
tctgcgcgctgacgtccgacgctccagg

SEQ ID NO: 27943 - DNA, 28 bp, synthetic construct
  source 1..28: mol_type = other DNA
agcgtcggacgtcagcgcgcagactcgg

SEQ ID NO: 27944 - DNA, 28 bp, synthetic construct
  source 1..28: mol_type = other DNA
agcgcgcagactcggcgcccgagcgcgg

SEQ ID NO: 27945 - DNA, 28 bp, synthetic construct
  source 1..28: mol_type = other DNA
tcggcgcccgagcgcggcgcgaagtcgg

SEQ ID NO: 27946 - DNA, 28 bp, synthetic construct
  source 1..28: mol_type = other DNA
gcgcccgagcgcggcgcgaagtcggcgg

SEQ ID NO: 27947 - DNA, 28 bp, synthetic construct
  source 1..28: mol_type = other DNA
ccgccgccgacttcgcgccgcgctcggg

SEQ ID NO: 27948 - DNA, 28 bp, synthetic construct
  source 1..28: mol_type = other DNA
cccgccgccgacttcgcgccgcgctcgg

SEQ ID NO: 27949 - DNA, 28 bp, synthetic construct
  source 1..28: mol_type = other DNA
cgagcgcggcgcgaagtcggcggcgggg

SEQ ID NO: 27950 - DNA, 28 bp, synthetic construct
  source 1..28: mol_type = other DNA
gcgcggcgcgaagtcggcggcggggcgg

SEQ ID NO: 27951 - DNA, 28 bp, synthetic construct
  source 1..28: mol_type = other DNA
cgcggcgcgaagtcggcggcggggcggg

SEQ ID NO: 27952 - DNA, 28 bp, synthetic construct
  source 1..28: mol_type = other DNA
gcggcgcgaagtcggcggcggggcgggg

SEQ ID NO: 27953 - DNA, 28 bp, synthetic construct
  source 1..28: mol_type = other DNA
gcgcgaagtcggcggcggggcggggcgg

SEQ ID NO: 27954 - DNA, 28 bp, synthetic construct
  source 1..28: mol_type = other DNA
cgcgaagtcggcggcggggcggggcggg

SEQ ID NO: 27955 - DNA, 28 bp, synthetic construct
  source 1..28: mol_type = other DNA
gcgaagtcggcggcggggcggggcgggg

SEQ ID NO: 27956 - DNA, 28 bp, synthetic construct
  source 1..28: mol_type = other DNA
cggcggcggggcggggcggggcgctcgg

SEQ ID NO: 27957 - DNA, 28 bp, synthetic construct
  source 1..28: mol_type = other DNA
ggcggcggggcggggcggggcgctcggg

SEQ ID NO: 27958 - DNA, 28 bp, synthetic construct
  source 1..28: mol_type = other DNA
gcggcggggcggggcggggcgctcgggg

SEQ ID NO: 27959 - DNA, 28 bp, synthetic construct
  source 1..28: mol_type = other DNA
cggcggggcggggcggggcgctcggggg

SEQ ID NO: 27960 - DNA, 28 bp, synthetic construct
  source 1..28: mol_type = other DNA
ggcggggcggggcggggcgctcgggggg

SEQ ID NO: 27961 - DNA, 28 bp, synthetic construct
  source 1..28: mol_type = other DNA
ggggcggggcggggcgctcggggggcgg

SEQ ID NO: 27962 - DNA, 28 bp, synthetic construct
  source 1..28: mol_type = other DNA
gggcggggcggggcgctcggggggcggg

SEQ ID NO: 27963 - DNA, 28 bp, synthetic construct
  source 1..28: mol_type = other DNA
ggcggggcggggcgctcggggggcgggg

SEQ ID NO: 27964 - DNA, 28 bp, synthetic construct
  source 1..28: mol_type = other DNA
ggcggggcgctcggggggcggggctcgg

SEQ ID NO: 27965 - DNA, 28 bp, synthetic construct
  source 1..28: mol_type = other DNA
gcggggcgctcggggggcggggctcggg

SEQ ID NO: 27966 - DNA, 28 bp, synthetic construct
  source 1..28: mol_type = other DNA
cggggcgctcggggggcggggctcgggg

SEQ ID NO: 27967 - DNA, 28 bp, synthetic construct
  source 1..28: mol_type = other DNA
tcggggggcggggctcggggtgcccagg

SEQ ID NO: 27968 - DNA, 28 bp, synthetic construct
  source 1..28: mol_type = other DNA
gggggcggggctcggggtgcccaggtgg

SEQ ID NO: 27969 - DNA, 28 bp, synthetic construct
  source 1..28: mol_type = other DNA
ggggcggggctcggggtgcccaggtggg

SEQ ID NO: 27970 - DNA, 28 bp, synthetic construct
  source 1..28: mol_type = other DNA
gcggggctcggggtgcccaggtgggagg

SEQ ID NO: 27971 - DNA, 28 bp, synthetic construct
  source 1..28: mol_type = other DNA
cggggctcggggtgcccaggtgggaggg

SEQ ID NO: 27972 - DNA, 28 bp, synthetic construct
  source 1..28: mol_type = other DNA
ggggctcggggtgcccaggtgggagggg

SEQ ID NO: 27973 - DNA, 28 bp, synthetic construct
  source 1..28: mol_type = other DNA
gggctcggggtgcccaggtgggaggggg

SEQ ID NO: 27974 - DNA, 28 bp, synthetic construct
  source 1..28: mol_type = other DNA
ctcggggtgcccaggtgggagggggcgg

SEQ ID NO: 27975 - DNA, 28 bp, synthetic construct
  source 1..28: mol_type = other DNA
tcggggtgcccaggtgggagggggcggg

SEQ ID NO: 27976 - DNA, 28 bp, synthetic construct
  source 1..28: mol_type = other DNA
cggggtgcccaggtgggagggggcgggg

SEQ ID NO: 27977 - DNA, 28 bp, synthetic construct
  source 1..28: mol_type = other DNA
tgcccaggtgggagggggcggggccagg

SEQ ID NO: 27978 - DNA, 28 bp, synthetic construct
  source 1..28: mol_type = other DNA
gcccaggtgggagggggcggggccaggg

SEQ ID NO: 27979 - DNA, 28 bp, synthetic construct
  source 1..28: mol_type = other DNA
cccaggtgggagggggcggggccagggg

SEQ ID NO: 27980 - DNA, 28 bp, synthetic construct
  source 1..28: mol_type = other DNA
tcccctggccccgccccctcccacctgg

SEQ ID NO: 27981 - DNA, 28 bp, synthetic construct
  source 1..28: mol_type = other DNA
gagggggcggggccaggggaccacccgg

SEQ ID NO: 27982 - DNA, 28 bp, synthetic construct
  source 1..28: mol_type = other DNA
ggggcggggccaggggaccacccggcgg

SEQ ID NO: 27983 - DNA, 28 bp, synthetic construct
  source 1..28: mol_type = other DNA
gggccaggggaccacccggcggccgtgg

SEQ ID NO: 27984 - DNA, 28 bp, synthetic construct
  source 1..28: mol_type = other DNA
ggaccacggccgccgggtggtcccctgg

SEQ ID NO: 27985 - DNA, 28 bp, synthetic construct
  source 1..28: mol_type = other DNA
gcgcgcagggaccacggccgccgggtgg

SEQ ID NO: 27986 - DNA, 28 bp, synthetic construct
  source 1..28: mol_type = other DNA
acccggcggccgtggtccctgcgcgcgg

SEQ ID NO: 27987 - DNA, 28 bp, synthetic construct
  source 1..28: mol_type = other DNA
gccgcgcgcagggaccacggccgccggg

SEQ ID NO: 27988 - DNA, 28 bp, synthetic construct
  source 1..28: mol_type = other DNA
tgccgcgcgcagggaccacggccgccgg

SEQ ID NO: 27989 - DNA, 28 bp, synthetic construct
  source 1..28: mol_type = other DNA
ggccgtggtccctgcgcgcggcacgagg

SEQ ID NO: 27990 - DNA, 28 bp, synthetic construct
  source 1..28: mol_type = other DNA
cacctcgtgccgcgcgcagggaccacgg

SEQ ID NO: 27991 - DNA, 28 bp, synthetic construct
  source 1..28: mol_type = other DNA
ggcggctcacctcgtgccgcgcgcaggg

SEQ ID NO: 27992 - DNA, 28 bp, synthetic construct
  source 1..28: mol_type = other DNA
gggcggctcacctcgtgccgcgcgcagg

SEQ ID NO: 27993 - DNA, 28 bp, synthetic construct
  source 1..28: mol_type = other DNA
gcgcggcacgaggtgagccgccccttgg

SEQ ID NO: 27994 - DNA, 28 bp, synthetic construct
  source 1..28: mol_type = other DNA
cgcggcacgaggtgagccgccccttggg

SEQ ID NO: 27995 - DNA, 28 bp, synthetic construct
  source 1..28: mol_type = other DNA
tgtcggaagacgcaagcccaaggggcgg

SEQ ID NO: 27996 - DNA, 28 bp, synthetic construct
  source 1..28: mol_type = other DNA
tcttgtcggaagacgcaagcccaagggg

SEQ ID NO: 27997 - DNA, 28 bp, synthetic construct
  source 1..28: mol_type = other DNA
ctcttgtcggaagacgcaagcccaaggg

SEQ ID NO: 27998 - DNA, 28 bp, synthetic construct
  source 1..28: mol_type = other DNA
tctcttgtcggaagacgcaagcccaagg

SEQ ID NO: 27999 - DNA, 28 bp, synthetic construct
  source 1..28: mol_type = other DNA
gggcttgcgtcttccgacaagagagagg

SEQ ID NO: 28000 - DNA, 28 bp, synthetic construct
  source 1..28: mol_type = other DNA
cttgcgtcttccgacaagagagaggcgg

SEQ ID NO: 28001 - DNA, 28 bp, synthetic construct
  source 1..28: mol_type = other DNA
gcgtcttccgacaagagagaggcggtgg

SEQ ID NO: 28002 - DNA, 28 bp, synthetic construct
  source 1..28: mol_type = other DNA
ccgacaagagagaggcggtggtccgtgg

SEQ ID NO: 28003 - DNA, 28 bp, synthetic construct
  source 1..28: mol_type = other DNA
cgacaagagagaggcggtggtccgtggg

SEQ ID NO: 28004 - DNA, 28 bp, synthetic construct
  source 1..28: mol_type = other DNA
gagaggcggtggtccgtgggtagcgcgg

SEQ ID NO: 28005 - DNA, 28 bp, synthetic construct
  source 1..28: mol_type = other DNA
agaggcggtggtccgtgggtagcgcggg

SEQ ID NO: 28006 - DNA, 28 bp, synthetic construct
  source 1..28: mol_type = other DNA
gaggcggtggtccgtgggtagcgcgggg

SEQ ID NO: 28007 - DNA, 28 bp, synthetic construct
  source 1..28: mol_type = other DNA
tggtccgtgggtagcgcggggttactgg

SEQ ID NO: 28008 - DNA, 28 bp, synthetic construct
  source 1..28: mol_type = other DNA
cattccagtaaccccgcgctacccacgg

SEQ ID NO: 28009 - DNA, 28 bp, synthetic construct
  source 1..28: mol_type = other DNA
cgtgggtagcgcggggttactggaatgg

SEQ ID NO: 28010 - DNA, 28 bp, synthetic construct
  source 1..28: mol_type = other DNA
gtgggtagcgcggggttactggaatggg

SEQ ID NO: 28011 - DNA, 28 bp, synthetic construct
  source 1..28: mol_type = other DNA
ggggttactggaatgggactccctgagg

SEQ ID NO: 28012 - DNA, 28 bp, synthetic construct
  source 1..28: mol_type = other DNA
ggcgacttctcaggggacttcctcaggg

SEQ ID NO: 28013 - DNA, 28 bp, synthetic construct
  source 1..28: mol_type = other DNA
cggcgacttctcaggggacttcctcagg

SEQ ID NO: 28014 - DNA, 28 bp, synthetic construct
  source 1..28: mol_type = other DNA
ctgaggaagtcccctgagaagtcgccgg

SEQ ID NO: 28015 - DNA, 28 bp, synthetic construct
  source 1..28: mol_type = other DNA
gcggagcgtgccggcgacttctcagggg

SEQ ID NO: 28016 - DNA, 28 bp, synthetic construct
  source 1..28: mol_type = other DNA
ggcggagcgtgccggcgacttctcaggg

SEQ ID NO: 28017 - DNA, 28 bp, synthetic construct
  source 1..28: mol_type = other DNA
aggcggagcgtgccggcgacttctcagg

SEQ ID NO: 28018 - DNA, 28 bp, synthetic construct
  source 1..28: mol_type = other DNA
aagcaagaaggaaggcggagcgtgccgg

SEQ ID NO: 28019 - DNA, 28 bp, synthetic construct
  source 1..28: mol_type = other DNA
gagaaatgggaagcaagaaggaaggcgg

SEQ ID NO: 28020 - DNA, 28 bp, synthetic construct
  source 1..28: mol_type = other DNA
aacgagaaatgggaagcaagaaggaagg

SEQ ID NO: 28021 - DNA, 28 bp, synthetic construct
  source 1..28: mol_type = other DNA
agaaaacgagaaatgggaagcaagaagg

SEQ ID NO: 28022 - DNA, 28 bp, synthetic construct
  source 1..28: mol_type = other DNA
gaaggctgagaagaaaacgagaaatggg

SEQ ID NO: 28023 - DNA, 28 bp, synthetic construct
  source 1..28: mol_type = other DNA
tgaaggctgagaagaaaacgagaaatgg

SEQ ID NO: 28024 - DNA, 28 bp, synthetic construct
  source 1..28: mol_type = other DNA
aatacagcactttaaaaaactatgaagg

SEQ ID NO: 28025 - DNA, 28 bp, synthetic construct
  source 1..28: mol_type = other DNA
ttgaatattattttaaacatcatctagg

SEQ ID NO: 28026 - DNA, 28 bp, synthetic construct
  source 1..28: mol_type = other DNA
ttaaacatcatctaggtcagattagcgg

SEQ ID NO: 28027 - DNA, 28 bp, synthetic construct
  source 1..28: mol_type = other DNA
tcagattagcggcctgtgaccaacttgg

SEQ ID NO: 28028 - DNA, 28 bp, synthetic construct
  source 1..28: mol_type = other DNA
aggaatttgtttccaagttggtcacagg

SEQ ID NO: 28029 - DNA, 28 bp, synthetic construct
  source 1..28: mol_type = other DNA
aagaatgaggaatttgtttccaagttgg

SEQ ID NO: 28030 - DNA, 28 bp, synthetic construct
  source 1..28: mol_type = other DNA
acaaattcctcattcttttctgccctgg

SEQ ID NO: 28031 - DNA, 28 bp, synthetic construct
  source 1..28: mol_type = other DNA
gctgacaccagggcagaaaagaatgagg

SEQ ID NO: 28032 - DNA, 28 bp, synthetic construct
  source 1..28: mol_type = other DNA
tgcaggcttacaggagctgacaccaggg

SEQ ID NO: 28033 - DNA, 28 bp, synthetic construct
  source 1..28: mol_type = other DNA
ctgcaggcttacaggagctgacaccagg

SEQ ID NO: 28034 - DNA, 28 bp, synthetic construct
  source 1..28: mol_type = other DNA
tttggcataaaatctgcaggcttacagg

SEQ ID NO: 28035 - DNA, 28 bp, synthetic construct
  source 1..28: mol_type = other DNA
gcggtttatttggcataaaatctgcagg

SEQ ID NO: 28036 - DNA, 28 bp, synthetic construct
  source 1..28: mol_type = other DNA
gcagattttatgccaaataaaccgctgg

SEQ ID NO: 28037 - DNA, 28 bp, synthetic construct
  source 1..28: mol_type = other DNA
atgccaaataaaccgctggagcaaaagg

SEQ ID NO: 28038 - DNA, 28 bp, synthetic construct
  source 1..28: mol_type = other DNA
tttccttttgctccagcggtttatttgg

SEQ ID NO: 28039 - DNA, 28 bp, synthetic construct
  source 1..28: mol_type = other DNA
aaataaaccgctggagcaaaaggaaagg

SEQ ID NO: 28040 - DNA, 28 bp, synthetic construct
  source 1..28: mol_type = other DNA
ctggctgcctttccttttgctccagcgg

SEQ ID NO: 28041 - DNA, 28 bp, synthetic construct
  source 1..28: mol_type = other DNA
aaaaggaaaggcagccagcctctcccgg

SEQ ID NO: 28042 - DNA, 28 bp, synthetic construct
  source 1..28: mol_type = other DNA
aaggcagccagcctctcccggaatttgg

SEQ ID NO: 28043 - DNA, 28 bp, synthetic construct
  source 1..28: mol_type = other DNA
aggcagccagcctctcccggaatttggg

SEQ ID NO: 28044 - DNA, 28 bp, synthetic construct
  source 1..28: mol_type = other DNA
gccagcctctcccggaatttgggagagg

SEQ ID NO: 28045 - DNA, 28 bp, synthetic construct
  source 1..28: mol_type = other DNA
ccctctcccaaattccgggagaggctgg

SEQ ID NO: 28046 - DNA, 28 bp, synthetic construct
  source 1..28: mol_type = other DNA
gtatccctctcccaaattccgggagagg

SEQ ID NO: 28047 - DNA, 28 bp, synthetic construct
  source 1..28: mol_type = other DNA
acaaggtatccctctcccaaattccggg

SEQ ID NO: 28048 - DNA, 28 bp, synthetic construct
  source 1..28: mol_type = other DNA
aacaaggtatccctctcccaaattccgg

SEQ ID NO: 28049 - DNA, 28 bp, synthetic construct
  source 1..28: mol_type = other DNA
taagttgtagaacgttttcttaacaagg

SEQ ID NO: 28050 - DNA, 28 bp, synthetic construct
  source 1..28: mol_type = other DNA
aactagtacgtttgtttggtaaaagagg

SEQ ID NO: 28051 - DNA, 28 bp, synthetic construct
  source 1..28: mol_type = other DNA
cttttaccaaacaaacgtactagttagg

SEQ ID NO: 28052 - DNA, 28 bp, synthetic construct
  source 1..28: mol_type = other DNA
ttttaccaaacaaacgtactagttaggg

SEQ ID NO: 28053 - DNA, 28 bp, synthetic construct
  source 1..28: mol_type = other DNA
gatttccctaactagtacgtttgtttgg

SEQ ID NO: 28054 - DNA, 28 bp, synthetic construct
  source 1..28: mol_type = other DNA
acgtttcttatgaagattatatagcagg

SEQ ID NO: 28055 - DNA, 28 bp, synthetic construct
  source 1..28: mol_type = other DNA
tatataatcttcataagaaacgtgaagg

SEQ ID NO: 28056 - DNA, 28 bp, synthetic construct
  source 1..28: mol_type = other DNA
atataatcttcataagaaacgtgaaggg

SEQ ID NO: 28057 - DNA, 28 bp, synthetic construct
  source 1..28: mol_type = other DNA
atcttcataagaaacgtgaagggttagg

SEQ ID NO: 28058 - DNA, 28 bp, synthetic construct
  source 1..28: mol_type = other DNA
cataagaaacgtgaagggttaggaaagg

SEQ ID NO: 28059 - DNA, 28 bp, synthetic construct
  source 1..28: mol_type = other DNA
aaggtttagccgtgctgtccagtattgg

SEQ ID NO: 28060 - DNA, 28 bp, synthetic construct
  source 1..28: mol_type = other DNA
aggtttagccgtgctgtccagtattggg

SEQ ID NO: 28061 - DNA, 28 bp, synthetic construct
  source 1..28: mol_type = other DNA
atttaaatcccaatactggacagcacgg

SEQ ID NO: 28062 - DNA, 28 bp, synthetic construct
  source 1..28: mol_type = other DNA
atatttaaaatttaaatcccaatactgg

SEQ ID NO: 28063 - DNA, 28 bp, synthetic construct
  source 1..28: mol_type = other DNA
tttaaatattaacttaattcctcagtgg

SEQ ID NO: 28064 - DNA, 28 bp, synthetic construct
  source 1..28: mol_type = other DNA
tcctcagtggcaccagccacatttcagg

SEQ ID NO: 28065 - DNA, 28 bp, synthetic construct
  source 1..28: mol_type = other DNA
acctgaaatgtggctggtgccactgagg

SEQ ID NO: 28066 - DNA, 28 bp, synthetic construct
  source 1..28: mol_type = other DNA
ggttatggcacacctgaaatgtggctgg

SEQ ID NO: 28067 - DNA, 28 bp, synthetic construct
  source 1..28: mol_type = other DNA
acatggttatggcacacctgaaatgtgg

SEQ ID NO: 28068 - DNA, 28 bp, synthetic construct
  source 1..28: mol_type = other DNA
atttcaggtgtgccataaccatgtatgg

SEQ ID NO: 28069 - DNA, 28 bp, synthetic construct
  source 1..28: mol_type = other DNA
gtgtgccataaccatgtatggctagtgg

SEQ ID NO: 28070 - DNA, 28 bp, synthetic construct
  source 1..28: mol_type = other DNA
agcagccactagccatacatggttatgg

SEQ ID NO: 28071 - DNA, 28 bp, synthetic construct
  source 1..28: mol_type = other DNA
ccacatagcagccactagccatacatgg

SEQ ID NO: 28072 - DNA, 28 bp, synthetic construct
  source 1..28: mol_type = other DNA
tttctatcatcgaagacagttcttttgg

SEQ ID NO: 28073 - DNA, 28 bp, synthetic construct
  source 1..28: mol_type = other DNA
cgaagacagttcttttggacagagccgg

SEQ ID NO: 28074 - DNA, 28 bp, synthetic construct
  source 1..28: mol_type = other DNA
gttcttttggacagagccggccgagagg

SEQ ID NO: 28075 - DNA, 28 bp, synthetic construct
  source 1..28: mol_type = other DNA
agccggccgagaggattacaatacttgg

SEQ ID NO: 28076 - DNA, 28 bp, synthetic construct
  source 1..28: mol_type = other DNA
gccggccgagaggattacaatacttggg

SEQ ID NO: 28077 - DNA, 28 bp, synthetic construct
  source 1..28: mol_type = other DNA
ccccaagtattgtaatcctctcggccgg

SEQ ID NO: 28078 - DNA, 28 bp, synthetic construct
  source 1..28: mol_type = other DNA
tctgccccaagtattgtaatcctctcgg

SEQ ID NO: 28079 - DNA, 28 bp, synthetic construct
  source 1..28: mol_type = other DNA
gggttttcattattttatgtgattaagg

SEQ ID NO: 28080 - DNA, 28 bp, synthetic construct
  source 1..28: mol_type = other DNA
acttttttttttttttttctggctaggg

SEQ ID NO: 28081 - DNA, 28 bp, synthetic construct
  source 1..28: mol_type = other DNA
aacttttttttttttttttctggctagg

SEQ ID NO: 28082 - DNA, 28 bp, synthetic construct
  source 1..28: mol_type = other DNA
tagccagaaaaaaaaaaaaaaaagttgg

SEQ ID NO: 28083 - DNA, 28 bp, synthetic construct
  source 1..28: mol_type = other DNA
tagccaacttttttttttttttttctgg

SEQ ID NO: 28084 - DNA, 28 bp, synthetic construct
  source 1..28: mol_type = other DNA
gaaaaaaaaaaaaaaaagttggctacgg

SEQ ID NO: 28085 - DNA, 28 bp, synthetic construct
  source 1..28: mol_type = other DNA
cttacatagtatgatttagagatacagg

SEQ ID NO: 28086 - DNA, 28 bp, synthetic construct
  source 1..28: mol_type = other DNA
cattagacattgtggggtctttcggggg

SEQ ID NO: 28087 - DNA, 28 bp, synthetic construct
  source 1..28: mol_type = other DNA
ccccgaaagaccccacaatgtctaatgg

SEQ ID NO: 28088 - DNA, 28 bp, synthetic construct
  source 1..28: mol_type = other DNA
accattagacattgtggggtctttcggg

SEQ ID NO: 28089 - DNA, 28 bp, synthetic construct
  source 1..28: mol_type = other DNA
gaccattagacattgtggggtctttcgg

SEQ ID NO: 28090 - DNA, 28 bp, synthetic construct
  source 1..28: mol_type = other DNA
agaccccacaatgtctaatggtccttgg

SEQ ID NO: 28091 - DNA, 28 bp, synthetic construct
  source 1..28: mol_type = other DNA
gaaccaaggaccattagacattgtgggg

SEQ ID NO: 28092 - DNA, 28 bp, synthetic construct
  source 1..28: mol_type = other DNA
agaaccaaggaccattagacattgtggg

SEQ ID NO: 28093 - DNA, 28 bp, synthetic construct
  source 1..28: mol_type = other DNA
cagaaccaaggaccattagacattgtgg

SEQ ID NO: 28094 - DNA, 28 bp, synthetic construct
  source 1..28: mol_type = other DNA
attcaatgacagaatttcagaaccaagg

SEQ ID NO: 28095 - DNA, 28 bp, synthetic construct
  source 1..28: mol_type = other DNA
cattgaatctgattattttgattaaagg

SEQ ID NO: 28096 - DNA, 28 bp, synthetic construct
  source 1..28: mol_type = other DNA
aatctgattattttgattaaaggcatgg

SEQ ID NO: 28097 - DNA, 28 bp, synthetic construct
  source 1..28: mol_type = other DNA
aatgcgaacattcacaggatattctggg

SEQ ID NO: 28098 - DNA, 28 bp, synthetic construct
  source 1..28: mol_type = other DNA
taatgcgaacattcacaggatattctgg

SEQ ID NO: 28099 - DNA, 28 bp, synthetic construct
  source 1..28: mol_type = other DNA
tgagcagactaatgcgaacattcacagg

SEQ ID NO: 28100 - DNA, 28 bp, synthetic construct
  source 1..28: mol_type = other DNA
tttgtagaacacagtattttttggttgg

SEQ ID NO: 28101 - DNA, 28 bp, synthetic construct
  source 1..28: mol_type = other DNA
aaccaaaaaatactgtgttctacaaagg

SEQ ID NO: 28102 - DNA, 28 bp, synthetic construct
  source 1..28: mol_type = other DNA
ctcctttgtagaacacagtattttttgg

SEQ ID NO: 28103 - DNA, 28 bp, synthetic construct
  source 1..28: mol_type = other DNA
caaaaaatactgtgttctacaaaggagg

SEQ ID NO: 28104 - DNA, 28 bp, synthetic construct
  source 1..28: mol_type = other DNA
tatcgccaagtattcagcatctctttgg

SEQ ID NO: 28105 - DNA, 28 bp, synthetic construct
  source 1..28: mol_type = other DNA
gaattccaaagagatgctgaatacttgg

SEQ ID NO: 28106 - DNA, 28 bp, synthetic construct
  source 1..28: mol_type = other DNA
tttggaattcatttgtcagcctctctgg

SEQ ID NO: 28107 - DNA, 28 bp, synthetic construct
  source 1..28: mol_type = other DNA
attcatttgtcagcctctctggttccgg

SEQ ID NO: 28108 - DNA, 28 bp, synthetic construct
  source 1..28: mol_type = other DNA
ttcatttgtcagcctctctggttccggg

SEQ ID NO: 28109 - DNA, 28 bp, synthetic construct
  source 1..28: mol_type = other DNA
gcaaatacagctcccggaaccagagagg

SEQ ID NO: 28110 - DNA, 28 bp, synthetic construct
  source 1..28: mol_type = other DNA
aactaagataggcaaatacagctcccgg

SEQ ID NO: 28111 - DNA, 28 bp, synthetic construct
  source 1..28: mol_type = other DNA
ttcgctgcactcagcaaactaagatagg

SEQ ID NO: 28112 - DNA, 28 bp, synthetic construct
  source 1..28: mol_type = other DNA
gagtgcagcgaagaatctagaacagtgg

SEQ ID NO: 28113 - DNA, 28 bp, synthetic construct
  source 1..28: mol_type = other DNA
agctcacactggatgcaaatgatgctgg

SEQ ID NO: 28114 - DNA, 28 bp, synthetic construct
  source 1..28: mol_type = other DNA
atttgcatttcaaagaagctcacactgg

SEQ ID NO: 28115 - DNA, 28 bp, synthetic construct
  source 1..28: mol_type = other DNA
gagcttctttgaaatgcaaatttgaagg

SEQ ID NO: 28116 - DNA, 28 bp, synthetic construct
  source 1..28: mol_type = other DNA
agtgatgtggttaacttcatgtggtagg

SEQ ID NO: 28117 - DNA, 28 bp, synthetic construct
  source 1..28: mol_type = other DNA
tttcagtgatgtggttaacttcatgtgg

SEQ ID NO: 28118 - DNA, 28 bp, synthetic construct
  source 1..28: mol_type = other DNA
ccacatcactgaaaaaaaagaaacatgg

SEQ ID NO: 28119 - DNA, 28 bp, synthetic construct
  source 1..28: mol_type = other DNA
aagaaacatggaaactgaattcacgagg

SEQ ID NO: 28120 - DNA, 28 bp, synthetic construct
  source 1..28: mol_type = other DNA
agaaacatggaaactgaattcacgaggg

SEQ ID NO: 28121 - DNA, 28 bp, synthetic construct
  source 1..28: mol_type = other DNA
ttgtaactatgcagttgcatgtgaacgg

SEQ ID NO: 28122 - DNA, 28 bp, synthetic construct
  source 1..28: mol_type = other DNA
tgataaagactcacctccccctgcttgg

SEQ ID NO: 28123 - DNA, 28 bp, synthetic construct
  source 1..28: mol_type = other DNA
gataaagactcacctccccctgcttggg

SEQ ID NO: 28124 - DNA, 28 bp, synthetic construct
  source 1..28: mol_type = other DNA
ataaagactcacctccccctgcttgggg

SEQ ID NO: 28125 - DNA, 28 bp, synthetic construct
  source 1..28: mol_type = other DNA
aagttcagcatccccaagcagggggagg

SEQ ID NO: 28126 - DNA, 28 bp, synthetic construct
  source 1..28: mol_type = other DNA
tccccctgcttggggatgctgaacttgg

SEQ ID NO: 28127 - DNA, 28 bp, synthetic construct
  source 1..28: mol_type = other DNA
tccaagttcagcatccccaagcaggggg

SEQ ID NO: 28128 - DNA, 28 bp, synthetic construct
  source 1..28: mol_type = other DNA
ctccaagttcagcatccccaagcagggg

SEQ ID NO: 28129 - DNA, 28 bp, synthetic construct
  source 1..28: mol_type = other DNA
tctccaagttcagcatccccaagcaggg

SEQ ID NO: 28130 - DNA, 28 bp, synthetic construct
  source 1..28: mol_type = other DNA
ctctccaagttcagcatccccaagcagg

SEQ ID NO: 28131 - DNA, 28 bp, synthetic construct
  source 1..28: mol_type = other DNA
ttggggatgctgaacttggagagcttgg

SEQ ID NO: 28132 - DNA, 28 bp, synthetic construct
  source 1..28: mol_type = other DNA
atgctgaacttggagagcttggccttgg

SEQ ID NO: 28133 - DNA, 28 bp, synthetic construct
  source 1..28: mol_type = other DNA
aacttggagagcttggccttggctctgg

SEQ ID NO: 28134 - DNA, 28 bp, synthetic construct
  source 1..28: mol_type = other DNA
tggagagcttggccttggctctggcagg

SEQ ID NO: 28135 - DNA, 28 bp, synthetic construct
  source 1..28: mol_type = other DNA
gcttggccttggctctggcaggctccgg

SEQ ID NO: 28136 - DNA, 28 bp, synthetic construct
  source 1..28: mol_type = other DNA
agcaagccggagcctgccagagccaagg

SEQ ID NO: 28137 - DNA, 28 bp, synthetic construct
  source 1..28: mol_type = other DNA
ttggctctggcaggctccggcttgctgg

SEQ ID NO: 28138 - DNA, 28 bp, synthetic construct
  source 1..28: mol_type = other DNA
ctctggcaggctccggcttgctggcagg

SEQ ID NO: 28139 - DNA, 28 bp, synthetic construct
  source 1..28: mol_type = other DNA
tctggcaggctccggcttgctggcaggg

SEQ ID NO: 28140 - DNA, 28 bp, synthetic construct
  source 1..28: mol_type = other DNA
tacaggggagtccctgccagcaagccgg

SEQ ID NO: 28141 - DNA, 28 bp, synthetic construct
  source 1..28: mol_type = other DNA
ccagcgtgcactgcacatcatacagggg

SEQ ID NO: 28142 - DNA, 28 bp, synthetic construct
  source 1..28: mol_type = other DNA
accagcgtgcactgcacatcatacaggg

SEQ ID NO: 28143 - DNA, 28 bp, synthetic construct
  source 1..28: mol_type = other DNA
aaccagcgtgcactgcacatcatacagg

SEQ ID NO: 28144 - DNA, 28 bp, synthetic construct
  source 1..28: mol_type = other DNA
tggtttccgaagacgacttcagcttagg

SEQ ID NO: 28145 - DNA, 28 bp, synthetic construct
  source 1..28: mol_type = other DNA
gagtctcctaagctgaagtcgtcttcgg

SEQ ID NO: 28146 - DNA, 28 bp, synthetic construct
  source 1..28: mol_type = other DNA
acgacttcagcttaggagactcatcagg

SEQ ID NO: 28147 - DNA, 28 bp, synthetic construct
  source 1..28: mol_type = other DNA
cgacttcagcttaggagactcatcaggg

SEQ ID NO: 28148 - DNA, 28 bp, synthetic construct
  source 1..28: mol_type = other DNA
gacttcagcttaggagactcatcagggg

SEQ ID NO: 28149 - DNA, 28 bp, synthetic construct
  source 1..28: mol_type = other DNA
aggagactcatcaggggcctgatcttgg

SEQ ID NO: 28150 - DNA, 28 bp, synthetic construct
  source 1..28: mol_type = other DNA
caggggcctgatcttggccgtccattgg

SEQ ID NO: 28151 - DNA, 28 bp, synthetic construct
  source 1..28: mol_type = other DNA
gtgaggccaatggacggccaagatcagg

SEQ ID NO: 28152 - DNA, 28 bp, synthetic construct
  source 1..28: mol_type = other DNA
tggccgtccattggcctcacatacgcgg

SEQ ID NO: 28153 - DNA, 28 bp, synthetic construct
  source 1..28: mol_type = other DNA
cgaccgcgtatgtgaggccaatggacgg

SEQ ID NO: 28154 - DNA, 28 bp, synthetic construct
  source 1..28: mol_type = other DNA
cgtccattggcctcacatacgcggtcgg

SEQ ID NO: 28155 - DNA, 28 bp, synthetic construct
  source 1..28: mol_type = other DNA
aaaccgaccgcgtatgtgaggccaatgg

SEQ ID NO: 28156 - DNA, 28 bp, synthetic construct
  source 1..28: mol_type = other DNA
ccagcagaaaccgaccgcgtatgtgagg

SEQ ID NO: 28157 - DNA, 28 bp, synthetic construct
  source 1..28: mol_type = other DNA
atacgcggtcggtttctgctggaccagg

SEQ ID NO: 28158 - DNA, 28 bp, synthetic construct
  source 1..28: mol_type = other DNA
gcggtcggtttctgctggaccaggctgg

SEQ ID NO: 28159 - DNA, 28 bp, synthetic construct
  source 1..28: mol_type = other DNA
cggtcggtttctgctggaccaggctggg

SEQ ID NO: 28160 - DNA, 28 bp, synthetic construct
  source 1..28: mol_type = other DNA
ctggaccaggctgggttttgaagctagg

SEQ ID NO: 28161 - DNA, 28 bp, synthetic construct
  source 1..28: mol_type = other DNA
tggaccaggctgggttttgaagctaggg

SEQ ID NO: 28162 - DNA, 28 bp, synthetic construct
  source 1..28: mol_type = other DNA
ccaggctgggttttgaagctagggatgg

SEQ ID NO: 28163 - DNA, 28 bp, synthetic construct
  source 1..28: mol_type = other DNA
ggctgggttttgaagctagggatggagg

SEQ ID NO: 28164 - DNA, 28 bp, synthetic construct
  source 1..28: mol_type = other DNA
acacagtgtccgctgctgctgtgcttgg

SEQ ID NO: 28165 - DNA, 28 bp, synthetic construct
  source 1..28: mol_type = other DNA
ccatggcggccaagcacagcagcagcgg

SEQ ID NO: 28166 - DNA, 28 bp, synthetic construct
  source 1..28: mol_type = other DNA
tgctgctgtgcttggccgccatggcagg

SEQ ID NO: 28167 - DNA, 28 bp, synthetic construct
  source 1..28: mol_type = other DNA
tgctgtgcttggccgccatggcaggtgg

SEQ ID NO: 28168 - DNA, 28 bp, synthetic construct
  source 1..28: mol_type = other DNA
ggccgccatggcaggtggcctctcctgg

SEQ ID NO: 28169 - DNA, 28 bp, synthetic construct
  source 1..28: mol_type = other DNA
gccgccatggcaggtggcctctcctggg

SEQ ID NO: 28170 - DNA, 28 bp, synthetic construct
  source 1..28: mol_type = other DNA
acccaggagaggccacctgccatggcgg

SEQ ID NO: 28171 - DNA, 28 bp, synthetic construct
  source 1..28: mol_type = other DNA
cagacccaggagaggccacctgccatgg

SEQ ID NO: 28172 - DNA, 28 bp, synthetic construct
  source 1..28: mol_type = other DNA
ggcaggtggcctctcctgggtctgaagg

SEQ ID NO: 28173 - DNA, 28 bp, synthetic construct
  source 1..28: mol_type = other DNA
ggaggtgggccttcagacccaggagagg

SEQ ID NO: 28174 - DNA, 28 bp, synthetic construct
  source 1..28: mol_type = other DNA
aatgtggaggtgggccttcagacccagg

SEQ ID NO: 28175 - DNA, 28 bp, synthetic construct
  source 1..28: mol_type = other DNA
ccaaacaagtgtgcaatgtggaggtggg

SEQ ID NO: 28176 - DNA, 28 bp, synthetic construct
  source 1..28: mol_type = other DNA
gccaaacaagtgtgcaatgtggaggtgg

SEQ ID NO: 28177 - DNA, 28 bp, synthetic construct
  source 1..28: mol_type = other DNA
cgggccaaacaagtgtgcaatgtggagg

SEQ ID NO: 28178 - DNA, 28 bp, synthetic construct
  source 1..28: mol_type = other DNA
cctcgggccaaacaagtgtgcaatgtgg

SEQ ID NO: 28179 - DNA, 28 bp, synthetic construct
  source 1..28: mol_type = other DNA
gatggtgttggcagacagcagcctcggg

SEQ ID NO: 28180 - DNA, 28 bp, synthetic construct
  source 1..28: mol_type = other DNA
agatggtgttggcagacagcagcctcgg

SEQ ID NO: 28181 - DNA, 28 bp, synthetic construct
  source 1..28: mol_type = other DNA
tgtctgccaacaccatctccaagcaagg

SEQ ID NO: 28182 - DNA, 28 bp, synthetic construct
  source 1..28: mol_type = other DNA
tcaggaccttgcttggagatggtgttgg

SEQ ID NO: 28183 - DNA, 28 bp, synthetic construct
  source 1..28: mol_type = other DNA
gctctctcaggaccttgcttggagatgg

SEQ ID NO: 28184 - DNA, 28 bp, synthetic construct
  source 1..28: mol_type = other DNA
aacagggctctctcaggaccttgcttgg

SEQ ID NO: 28185 - DNA, 28 bp, synthetic construct
  source 1..28: mol_type = other DNA
caactcagcacaacagggctctctcagg

SEQ ID NO: 28186 - DNA, 28 bp, synthetic construct
  source 1..28: mol_type = other DNA
ctgagagagccctgttgtgctgagttgg

SEQ ID NO: 28187 - DNA, 28 bp, synthetic construct
  source 1..28: mol_type = other DNA
cttcttcttccaactcagcacaacaggg

SEQ ID NO: 28188 - DNA, 28 bp, synthetic construct
  source 1..28: mol_type = other DNA
tcttcttcttccaactcagcacaacagg

SEQ ID NO: 28189 - DNA, 28 bp, synthetic construct
  source 1..28: mol_type = other DNA
tgtgctgagttggaagaagaagaagagg

SEQ ID NO: 28190 - DNA, 28 bp, synthetic construct
  source 1..28: mol_type = other DNA
ttggaagaagaagaagaggaagataagg

SEQ ID NO: 28191 - DNA, 28 bp, synthetic construct
  source 1..28: mol_type = other DNA
gaagaagaagaggaagataaggatgagg

SEQ ID NO: 28192 - DNA, 28 bp, synthetic construct
  source 1..28: mol_type = other DNA
aagaagaagaggaagataaggatgaggg

SEQ ID NO: 28193 - DNA, 28 bp, synthetic construct
  source 1..28: mol_type = other DNA
agaagaagaggaagataaggatgagggg

SEQ ID NO: 28194 - DNA, 28 bp, synthetic construct
  source 1..28: mol_type = other DNA
gaagaagaggaagataaggatgaggggg

SEQ ID NO: 28195 - DNA, 28 bp, synthetic construct
  source 1..28: mol_type = other DNA
aagaagaggaagataaggatgagggggg

SEQ ID NO: 28196 - DNA, 28 bp, synthetic construct
  source 1..28: mol_type = other DNA
ataaggatgaggggggtcgacacatagg

SEQ ID NO: 28197 - DNA, 28 bp, synthetic construct
  source 1..28: mol_type = other DNA
taaggatgaggggggtcgacacataggg

SEQ ID NO: 28198 - DNA, 28 bp, synthetic construct
  source 1..28: mol_type = other DNA
attttcttttttcattatagttctctgg

SEQ ID NO: 28199 - DNA, 28 bp, synthetic construct
  source 1..28: mol_type = other DNA
ttttcttttttcattatagttctctggg

SEQ ID NO: 28200 - DNA, 28 bp, synthetic construct
  source 1..28: mol_type = other DNA
acagagagcaagtaagcacaggcacagg

SEQ ID NO: 28201 - DNA, 28 bp, synthetic construct
  source 1..28: mol_type = other DNA
gtgcctgtgcttacttgctctctgttgg

SEQ ID NO: 28202 - DNA, 28 bp, synthetic construct
  source 1..28: mol_type = other DNA
cggccaacagagagcaagtaagcacagg

SEQ ID NO: 28203 - DNA, 28 bp, synthetic construct
  source 1..28: mol_type = other DNA
ttacttgctctctgttggccgtcagagg

SEQ ID NO: 28204 - DNA, 28 bp, synthetic construct
  source 1..28: mol_type = other DNA
tacttgctctctgttggccgtcagaggg

SEQ ID NO: 28205 - DNA, 28 bp, synthetic construct
  source 1..28: mol_type = other DNA
ttgctctctgttggccgtcagagggtgg

SEQ ID NO: 28206 - DNA, 28 bp, synthetic construct
  source 1..28: mol_type = other DNA
tgctctctgttggccgtcagagggtggg

SEQ ID NO: 28207 - DNA, 28 bp, synthetic construct
  source 1..28: mol_type = other DNA
agaaggctgggcacccaccctctgacgg

SEQ ID NO: 28208 - DNA, 28 bp, synthetic construct
  source 1..28: mol_type = other DNA
aggcactatgggctggcagaaggctggg

SEQ ID NO: 28209 - DNA, 28 bp, synthetic construct
  source 1..28: mol_type = other DNA
gaggcactatgggctggcagaaggctgg

SEQ ID NO: 28210 - DNA, 28 bp, synthetic construct
  source 1..28: mol_type = other DNA
aagagaggcactatgggctggcagaagg

SEQ ID NO: 28211 - DNA, 28 bp, synthetic construct
  source 1..28: mol_type = other DNA
gcagagtaagagaggcactatgggctgg

SEQ ID NO: 28212 - DNA, 28 bp, synthetic construct
  source 1..28: mol_type = other DNA
tgcagcagagtaagagaggcactatggg

SEQ ID NO: 28213 - DNA, 28 bp, synthetic construct
  source 1..28: mol_type = other DNA
gtgcagcagagtaagagaggcactatgg

SEQ ID NO: 28214 - DNA, 28 bp, synthetic construct
  source 1..28: mol_type = other DNA
atagtgcctctcttactctgctgcacgg

SEQ ID NO: 28215 - DNA, 28 bp, synthetic construct
  source 1..28: mol_type = other DNA
tagtgcctctcttactctgctgcacggg

SEQ ID NO: 28216 - DNA, 28 bp, synthetic construct
  source 1..28: mol_type = other DNA
agtgcctctcttactctgctgcacgggg

SEQ ID NO: 28217 - DNA, 28 bp, synthetic construct
  source 1..28: mol_type = other DNA
ctgtccccgtgcagcagagtaagagagg

SEQ ID NO: 28218 - DNA, 28 bp, synthetic construct
  source 1..28: mol_type = other DNA
tactctgctgcacggggacagctgctgg

SEQ ID NO: 28219 - DNA, 28 bp, synthetic construct
  source 1..28: mol_type = other DNA
tgctgcacggggacagctgctggtgtgg

SEQ ID NO: 28220 - DNA, 28 bp, synthetic construct
  source 1..28: mol_type = other DNA
gaagttgtagtgctacagatagacgagg

SEQ ID NO: 28221 - DNA, 28 bp, synthetic construct
  source 1..28: mol_type = other DNA
aagttgtagtgctacagatagacgaggg

SEQ ID NO: 28222 - DNA, 28 bp, synthetic construct
  source 1..28: mol_type = other DNA
tgtagtgctacagatagacgagggctgg

SEQ ID NO: 28223 - DNA, 28 bp, synthetic construct
  source 1..28: mol_type = other DNA
gctacagatagacgagggctggttctgg

SEQ ID NO: 28224 - DNA, 28 bp, synthetic construct
  source 1..28: mol_type = other DNA
ctacagatagacgagggctggttctggg

SEQ ID NO: 28225 - DNA, 28 bp, synthetic construct
  source 1..28: mol_type = other DNA
caaaatgttcatcgatcttgttcacagg

SEQ ID NO: 28226 - DNA, 28 bp, synthetic construct
  source 1..28: mol_type = other DNA
catcgatcttgttcacaggagtctgagg

SEQ ID NO: 28227 - DNA, 28 bp, synthetic construct
  source 1..28: mol_type = other DNA
tgttcacaggagtctgaggaaccccagg

SEQ ID NO: 28228 - DNA, 28 bp, synthetic construct
  source 1..28: mol_type = other DNA
acaggagtctgaggaaccccaggtttgg

SEQ ID NO: 28229 - DNA, 28 bp, synthetic construct
  source 1..28: mol_type = other DNA
caggagtctgaggaaccccaggtttggg

SEQ ID NO: 28230 - DNA, 28 bp, synthetic construct
  source 1..28: mol_type = other DNA
catctcgttggagttcccaaacctgggg

SEQ ID NO: 28231 - DNA, 28 bp, synthetic construct
  source 1..28: mol_type = other DNA
tcatctcgttggagttcccaaacctggg

SEQ ID NO: 28232 - DNA, 28 bp, synthetic construct
  source 1..28: mol_type = other DNA
gtcatctcgttggagttcccaaacctgg

SEQ ID NO: 28233 - DNA, 28 bp, synthetic construct
  source 1..28: mol_type = other DNA
ggaactccaacgagatgactctgattgg

SEQ ID NO: 28234 - DNA, 28 bp, synthetic construct
  source 1..28: mol_type = other DNA
atagatccaatcagagtcatctcgttgg

SEQ ID NO: 28235 - DNA, 28 bp, synthetic construct
  source 1..28: mol_type = other DNA
ttcatcataattgcctaaagtgttctgg

SEQ ID NO: 28236 - DNA, 28 bp, synthetic construct
  source 1..28: mol_type = other DNA
ataattgcctaaagtgttctggatccgg

SEQ ID NO: 28237 - DNA, 28 bp, synthetic construct
  source 1..28: mol_type = other DNA
ttgcctaaagtgttctggatccggttgg

SEQ ID NO: 28238 - DNA, 28 bp, synthetic construct
  source 1..28: mol_type = other DNA
tctccaaccggatccagaacactttagg

SEQ ID NO: 28239 - DNA, 28 bp, synthetic construct
  source 1..28: mol_type = other DNA
taacaagggggatgaactctccaaccgg

SEQ ID NO: 28240 - DNA, 28 bp, synthetic construct
  source 1..28: mol_type = other DNA
ggagagttcatcccccttgttagtctgg

SEQ ID NO: 28241 - DNA, 28 bp, synthetic construct
  source 1..28: mol_type = other DNA
tttttctttctccagactaacaaggggg

SEQ ID NO: 28242 - DNA, 28 bp, synthetic construct
  source 1..28: mol_type = other DNA
gtttttctttctccagactaacaagggg

SEQ ID NO: 28243 - DNA, 28 bp, synthetic construct
  source 1..28: mol_type = other DNA
tgtttttctttctccagactaacaaggg

SEQ ID NO: 28244 - DNA, 28 bp, synthetic construct
  source 1..28: mol_type = other DNA
gtgtttttctttctccagactaacaagg

SEQ ID NO: 28245 - DNA, 28 bp, synthetic construct
  source 1..28: mol_type = other DNA
gtttctgttgtctctaacaatagcgtgg

SEQ ID NO: 28246 - DNA, 28 bp, synthetic construct
  source 1..28: mol_type = other DNA
ctattgttagagacaacagaaacaccgg

SEQ ID NO: 28247 - DNA, 28 bp, synthetic construct
  source 1..28: mol_type = other DNA
aacagaaacaccggagataatcaacagg

SEQ ID NO: 28248 - DNA, 28 bp, synthetic construct
  source 1..28: mol_type = other DNA
gataagggcacctgttgattatctccgg

SEQ ID NO: 28249 - DNA, 28 bp, synthetic construct
  source 1..28: mol_type = other DNA
aggtgcccttatcaatcacagagccagg

SEQ ID NO: 28250 - DNA, 28 bp, synthetic construct
  source 1..28: mol_type = other DNA
ggtgcccttatcaatcacagagccaggg

SEQ ID NO: 28251 - DNA, 28 bp, synthetic construct
  source 1..28: mol_type = other DNA
acaaccctggctctgtgattgataaggg

SEQ ID NO: 28252 - DNA, 28 bp, synthetic construct
  source 1..28: mol_type = other DNA
gacaaccctggctctgtgattgataagg

SEQ ID NO: 28253 - DNA, 28 bp, synthetic construct
  source 1..28: mol_type = other DNA
gctctcattctgcatgtgacaaccctgg

SEQ ID NO: 28254 - DNA, 28 bp, synthetic construct
  source 1..28: mol_type = other DNA
ctgcatcttctgtctgttcagcccaggg

SEQ ID NO: 28255 - DNA, 28 bp, synthetic construct
  source 1..28: mol_type = other DNA
actgcatcttctgtctgttcagcccagg

SEQ ID NO: 28256 - DNA, 28 bp, synthetic construct
  source 1..28: mol_type = other DNA
aacagacagaagatgcagtcaagtttgg

SEQ ID NO: 28257 - DNA, 28 bp, synthetic construct
  source 1..28: mol_type = other DNA
gacagaagatgcagtcaagtttggtcgg

SEQ ID NO: 28258 - DNA, 28 bp, synthetic construct
  source 1..28: mol_type = other DNA
tttggtcggccaattcttttagtcaagg

SEQ ID NO: 28259 - DNA, 28 bp, synthetic construct
  source 1..28: mol_type = other DNA
tgacggtggccttgactaaaagaattgg

SEQ ID NO: 28260 - DNA, 28 bp, synthetic construct
  source 1..28: mol_type = other DNA
ttcttttagtcaaggccaccgtcacagg

SEQ ID NO: 28261 - DNA, 28 bp, synthetic construct
  source 1..28: mol_type = other DNA
tcttttagtcaaggccaccgtcacaggg

SEQ ID NO: 28262 - DNA, 28 bp, synthetic construct
  source 1..28: mol_type = other DNA
ttgtttctctcactccctgtgacggtgg

SEQ ID NO: 28263 - DNA, 28 bp, synthetic construct
  source 1..28: mol_type = other DNA
cacttgtttctctcactccctgtgacgg

SEQ ID NO: 28264 - DNA, 28 bp, synthetic construct
  source 1..28: mol_type = other DNA
acagggagtgagagaaacaagtgagagg

SEQ ID NO: 28265 - DNA, 28 bp, synthetic construct
  source 1..28: mol_type = other DNA
aacaactgaaaaccatctaccttgtagg

SEQ ID NO: 28266 - DNA, 28 bp, synthetic construct
  source 1..28: mol_type = other DNA
acaactgaaaaccatctaccttgtaggg

SEQ ID NO: 28267 - DNA, 28 bp, synthetic construct
  source 1..28: mol_type = other DNA
tcttcagtgagccctacaaggtagatgg

SEQ ID NO: 28268 - DNA, 28 bp, synthetic construct
  source 1..28: mol_type = other DNA
tactctctcttcagtgagccctacaagg

SEQ ID NO: 28269 - DNA, 28 bp, synthetic construct
  source 1..28: mol_type = other DNA
gaaatcaagaaactcaacaggatgatgg

SEQ ID NO: 28270 - DNA, 28 bp, synthetic construct
  source 1..28: mol_type = other DNA
gaaagaagaaatcaagaaactcaacagg

SEQ ID NO: 28271 - DNA, 28 bp, synthetic construct
  source 1..28: mol_type = other DNA
ctttcctccgtaatgcatttctatctgg

SEQ ID NO: 28272 - DNA, 28 bp, synthetic construct
  source 1..28: mol_type = other DNA
tgaaccagatagaaatgcattacggagg

SEQ ID NO: 28273 - DNA, 28 bp, synthetic construct
  source 1..28: mol_type = other DNA
ctatgaaccagatagaaatgcattacgg

SEQ ID NO: 28274 - DNA, 28 bp, synthetic construct
  source 1..28: mol_type = other DNA
ctatctggttcatagacactgcatcagg

SEQ ID NO: 28275 - DNA, 28 bp, synthetic construct
  source 1..28: mol_type = other DNA
ggctttacagtttaatttgtgtgtgtgg

SEQ ID NO: 28276 - DNA, 28 bp, synthetic construct
  source 1..28: mol_type = other DNA
tctgcactcacacaagtgttacattggg

SEQ ID NO: 28277 - DNA, 28 bp, synthetic construct
  source 1..28: mol_type = other DNA
ttctgcactcacacaagtgttacattgg

SEQ ID NO: 28278 - DNA, 28 bp, synthetic construct
  source 1..28: mol_type = other DNA
taacacttgtgtgagtgcagaagtctgg

SEQ ID NO: 28279 - DNA, 28 bp, synthetic construct
  source 1..28: mol_type = other DNA
tgtgtgagtgcagaagtctggttcgtgg

SEQ ID NO: 28280 - DNA, 28 bp, synthetic construct
  source 1..28: mol_type = other DNA
tgcagaagtctggttcgtggacaaatgg

SEQ ID NO: 28281 - DNA, 28 bp, synthetic construct
  source 1..28: mol_type = other DNA
acaaatggtgatgacaacaagaacatgg

SEQ ID NO: 28282 - DNA, 28 bp, synthetic construct
  source 1..28: mol_type = other DNA
gtcaacccaaccagacacacaagactgg

SEQ ID NO: 28283 - DNA, 28 bp, synthetic construct
  source 1..28: mol_type = other DNA
tcacaccagtcttgtgtgtctggttggg

SEQ ID NO: 28284 - DNA, 28 bp, synthetic construct
  source 1..28: mol_type = other DNA
atcacaccagtcttgtgtgtctggttgg

SEQ ID NO: 28285 - DNA, 28 bp, synthetic construct
  source 1..28: mol_type = other DNA
gtgcatcacaccagtcttgtgtgtctgg

SEQ ID NO: 28286 - DNA, 28 bp, synthetic construct
  source 1..28: mol_type = other DNA
cacaagactggtgtgatgcacgaagtgg

SEQ ID NO: 28287 - DNA, 28 bp, synthetic construct
  source 1..28: mol_type = other DNA
atgcacgaagtggcctcatgtaagatgg

SEQ ID NO: 28288 - DNA, 28 bp, synthetic construct
  source 1..28: mol_type = other DNA
gaagtggcctcatgtaagatggagcagg

SEQ ID NO: 28289 - DNA, 28 bp, synthetic construct
  source 1..28: mol_type = other DNA
tggcctcatgtaagatggagcaggcagg

SEQ ID NO: 28290 - DNA, 28 bp, synthetic construct
  source 1..28: mol_type = other DNA
cctcatgtaagatggagcaggcaggtgg

SEQ ID NO: 28291 - DNA, 28 bp, synthetic construct
  source 1..28: mol_type = other DNA
gcaggtggtcattgagaatgatttctgg

SEQ ID NO: 28292 - DNA, 28 bp, synthetic construct
  source 1..28: mol_type = other DNA
caggtggtcattgagaatgatttctggg

SEQ ID NO: 28293 - DNA, 28 bp, synthetic construct
  source 1..28: mol_type = other DNA
gagaatgatttctgggcttctcagaagg

SEQ ID NO: 28294 - DNA, 28 bp, synthetic construct
  source 1..28: mol_type = other DNA
gcaggaggtattattttgggcatggggg

SEQ ID NO: 28295 - DNA, 28 bp, synthetic construct
  source 1..28: mol_type = other DNA
tgcaggaggtattattttgggcatgggg

SEQ ID NO: 28296 - DNA, 28 bp, synthetic construct
  source 1..28: mol_type = other DNA
atgcaggaggtattattttgggcatggg

SEQ ID NO: 28297 - DNA, 28 bp, synthetic construct
  source 1..28: mol_type = other DNA
gatgcaggaggtattattttgggcatgg

SEQ ID NO: 28298 - DNA, 28 bp, synthetic construct
  source 1..28: mol_type = other DNA
cagcagatgcaggaggtattattttggg

SEQ ID NO: 28299 - DNA, 28 bp, synthetic construct
  source 1..28: mol_type = other DNA
ccagcagatgcaggaggtattattttgg

SEQ ID NO: 28300 - DNA, 28 bp, synthetic construct
  source 1..28: mol_type = other DNA
tcagtcatcagccagcagatgcaggagg

SEQ ID NO: 28301 - DNA, 28 bp, synthetic construct
  source 1..28: mol_type = other DNA
atttcagtcatcagccagcagatgcagg

SEQ ID NO: 28302 - DNA, 28 bp, synthetic construct
  source 1..28: mol_type = other DNA
ttccacaactagagagtcattcctctgg

SEQ ID NO: 28303 - DNA, 28 bp, synthetic construct
  source 1..28: mol_type = other DNA
aaccagaggaatgactctctagttgtgg

SEQ ID NO: 28304 - DNA, 28 bp, synthetic construct
  source 1..28: mol_type = other DNA
caggggtgaagacatcttaaaccagagg

SEQ ID NO: 28305 - DNA, 28 bp, synthetic construct
  source 1..28: mol_type = other DNA
cttgtggtgtttatatttcttgcagggg

SEQ ID NO: 28306 - DNA, 28 bp, synthetic construct
  source 1..28: mol_type = other DNA
tcttgtggtgtttatatttcttgcaggg

SEQ ID NO: 28307 - DNA, 28 bp, synthetic construct
  source 1..28: mol_type = other DNA
ttcttgtggtgtttatatttcttgcagg

SEQ ID NO: 28308 - DNA, 28 bp, synthetic construct
  source 1..28: mol_type = other DNA
aggtttaaagtgtttcagcttcttgtgg

SEQ ID NO: 28309 - DNA, 28 bp, synthetic construct
  source 1..28: mol_type = other DNA
cacgctaagatactcaaggctaatcagg

SEQ ID NO: 28310 - DNA, 28 bp, synthetic construct
  source 1..28: mol_type = other DNA
agactcatgcacgctaagatactcaagg

SEQ ID NO: 28311 - DNA, 28 bp, synthetic construct
  source 1..28: mol_type = other DNA
ctgtcagcatattttccagaagccgagg

SEQ ID NO: 28312 - DNA, 28 bp, synthetic construct
  source 1..28: mol_type = other DNA
tgtcagcatattttccagaagccgaggg

SEQ ID NO: 28313 - DNA, 28 bp, synthetic construct
  source 1..28: mol_type = other DNA
gtcagcatattttccagaagccgagggg

SEQ ID NO: 28314 - DNA, 28 bp, synthetic construct
  source 1..28: mol_type = other DNA
tcttggattctttcccctcggcttctgg

SEQ ID NO: 28315 - DNA, 28 bp, synthetic construct
  source 1..28: mol_type = other DNA
gccgaggggaaagaatccaagatcccgg

SEQ ID NO: 28316 - DNA, 28 bp, synthetic construct
  source 1..28: mol_type = other DNA
tcaaagctatgcagagtaaactctcagg

SEQ ID NO: 28317 - DNA, 28 bp, synthetic construct
  source 1..28: mol_type = other DNA
ctgcagtaatgatgaagacaagctaagg

SEQ ID NO: 28318 - DNA, 28 bp, synthetic construct
  source 1..28: mol_type = other DNA
acaagctaaggtaatctaaaacaacagg

SEQ ID NO: 28319 - DNA, 28 bp, synthetic construct
  source 1..28: mol_type = other DNA
caagaggaagataattgatgataaaagg

SEQ ID NO: 28320 - DNA, 28 bp, synthetic construct
  source 1..28: mol_type = other DNA
cttttatcatcaattatcttcctcttgg

SEQ ID NO: 28321 - DNA, 28 bp, synthetic construct
  source 1..28: mol_type = other DNA
acataatttttcaactgctgccaagagg

SEQ ID NO: 28322 - DNA, 28 bp, synthetic construct
  source 1..28: mol_type = other DNA
aaaaattatgttttactcaaaagtcagg

SEQ ID NO: 28323 - DNA, 28 bp, synthetic construct
  source 1..28: mol_type = other DNA
tatttatacaacacttgaactgtgttgg

SEQ ID NO: 28324 - DNA, 28 bp, synthetic construct
  source 1..28: mol_type = other DNA
atttatacaacacttgaactgtgttggg

SEQ ID NO: 28325 - DNA, 28 bp, synthetic construct
  source 1..28: mol_type = other DNA
ttgggtgtcagcgtgttagccactgtgg

SEQ ID NO: 28326 - DNA, 28 bp, synthetic construct
  source 1..28: mol_type = other DNA
aacagcagaatttgaaattccacagtgg

SEQ ID NO: 28327 - DNA, 28 bp, synthetic construct
  source 1..28: mol_type = other DNA
agtacccgagagttgactctgagagtgg

SEQ ID NO: 28328 - DNA, 28 bp, synthetic construct
  source 1..28: mol_type = other DNA
aagaccactctcagagtcaactctcggg

SEQ ID NO: 28329 - DNA, 28 bp, synthetic construct
  source 1..28: mol_type = other DNA
gaagaccactctcagagtcaactctcgg

SEQ ID NO: 28330 - DNA, 28 bp, synthetic construct
  source 1..28: mol_type = other DNA
agtggtcttctaataactgtattcttgg

SEQ ID NO: 28331 - DNA, 28 bp, synthetic construct
  source 1..28: mol_type = other DNA
gcactgagctaaaacatctcattttagg

SEQ ID NO: 28332 - DNA, 28 bp, synthetic construct
  source 1..28: mol_type = other DNA
tcagtgccaagagtgtgaaaacacatgg

SEQ ID NO: 28333 - DNA, 28 bp, synthetic construct
  source 1..28: mol_type = other DNA
cagtgccaagagtgtgaaaacacatggg

SEQ ID NO: 28334 - DNA, 28 bp, synthetic construct
  source 1..28: mol_type = other DNA
agtgccaagagtgtgaaaacacatgggg

SEQ ID NO: 28335 - DNA, 28 bp, synthetic construct
  source 1..28: mol_type = other DNA
gtgccaagagtgtgaaaacacatggggg

SEQ ID NO: 28336 - DNA, 28 bp, synthetic construct
  source 1..28: mol_type = other DNA
atgcccccatgtgttttcacactcttgg

SEQ ID NO: 28337 - DNA, 28 bp, synthetic construct
  source 1..28: mol_type = other DNA
acatgggggcattacattagaaacctgg

SEQ ID NO: 28338 - DNA, 28 bp, synthetic construct
  source 1..28: mol_type = other DNA
catgggggcattacattagaaacctggg

SEQ ID NO: 28339 - DNA, 28 bp, synthetic construct
  source 1..28: mol_type = other DNA
aaaatgatattaattgacaggtcccagg

SEQ ID NO: 28340 - DNA, 28 bp, synthetic construct
  source 1..28: mol_type = other DNA
ttggaggaaaatgatattaattgacagg

SEQ ID NO: 28341 - DNA, 28 bp, synthetic construct
  source 1..28: mol_type = other DNA
tctggatgtattttcttcatgttggagg

SEQ ID NO: 28342 - DNA, 28 bp, synthetic construct
  source 1..28: mol_type = other DNA
agctctggatgtattttcttcatgttgg

SEQ ID NO: 28343 - DNA, 28 bp, synthetic construct
  source 1..28: mol_type = other DNA
atccagagctcagtcttctcatttatgg

SEQ ID NO: 28344 - DNA, 28 bp, synthetic construct
  source 1..28: mol_type = other DNA
ttccataaatgagaagactgagctctgg

SEQ ID NO: 28345 - DNA, 28 bp, synthetic construct
  source 1..28: mol_type = other DNA
gagctcagtcttctcatttatggaatgg

SEQ ID NO: 28346 - DNA, 28 bp, synthetic construct
  source 1..28: mol_type = other DNA
agctcagtcttctcatttatggaatggg

SEQ ID NO: 28347 - DNA, 28 bp, synthetic construct
  source 1..28: mol_type = other DNA
gctcagtcttctcatttatggaatgggg

SEQ ID NO: 28348 - DNA, 28 bp, synthetic construct
  source 1..28: mol_type = other DNA
gcctttcatagttgtcttttagaccagg

SEQ ID NO: 28349 - DNA, 28 bp, synthetic construct
  source 1..28: mol_type = other DNA
tcctggtctaaaagacaactatgaaagg

SEQ ID NO: 28350 - DNA, 28 bp, synthetic construct
  source 1..28: mol_type = other DNA
ggtgcttcttatacattatctttcctgg

SEQ ID NO: 28351 - DNA, 28 bp, synthetic construct
  source 1..28: mol_type = other DNA
gaagcacctagaatcatctttgacatgg

SEQ ID NO: 28352 - DNA, 28 bp, synthetic construct
  source 1..28: mol_type = other DNA
aagcacctagaatcatctttgacatggg

SEQ ID NO: 28353 - DNA, 28 bp, synthetic construct
  source 1..28: mol_type = other DNA
agcacctagaatcatctttgacatgggg

SEQ ID NO: 28354 - DNA, 28 bp, synthetic construct
  source 1..28: mol_type = other DNA
acctagaatcatctttgacatggggtgg

SEQ ID NO: 28355 - DNA, 28 bp, synthetic construct
  source 1..28: mol_type = other DNA
cctagaatcatctttgacatggggtggg

SEQ ID NO: 28356 - DNA, 28 bp, synthetic construct
  source 1..28: mol_type = other DNA
tttcagggatatgtctcatcataatagg

SEQ ID NO: 28357 - DNA, 28 bp, synthetic construct
  source 1..28: mol_type = other DNA
agacactcaaagggactctttttcaggg

SEQ ID NO: 28358 - DNA, 28 bp, synthetic construct
  source 1..28: mol_type = other DNA
aagacactcaaagggactctttttcagg

SEQ ID NO: 28359 - DNA, 28 bp, synthetic construct
  source 1..28: mol_type = other DNA
gtccctttgagtgtcttcgtctttccgg

SEQ ID NO: 28360 - DNA, 28 bp, synthetic construct
  source 1..28: mol_type = other DNA
agccggaaagacgaagacactcaaaggg

SEQ ID NO: 28361 - DNA, 28 bp, synthetic construct
  source 1..28: mol_type = other DNA
cagccggaaagacgaagacactcaaagg

SEQ ID NO: 28362 - DNA, 28 bp, synthetic construct
  source 1..28: mol_type = other DNA
ttcttgaatcagcagatgattcagccgg

SEQ ID NO: 28363 - DNA, 28 bp, synthetic construct
  source 1..28: mol_type = other DNA
ctgaatcatctgctgattcaagaagagg

SEQ ID NO: 28364 - DNA, 28 bp, synthetic construct
  source 1..28: mol_type = other DNA
aatcatctgctgattcaagaagaggagg

SEQ ID NO: 28365 - DNA, 28 bp, synthetic construct
  source 1..28: mol_type = other DNA
aggaggccatatgcagacagcacaaagg

SEQ ID NO: 28366 - DNA, 28 bp, synthetic construct
  source 1..28: mol_type = other DNA
ggaggccatatgcagacagcacaaaggg

SEQ ID NO: 28367 - DNA, 28 bp, synthetic construct
  source 1..28: mol_type = other DNA
gagttccctttgtgctgtctgcatatgg

SEQ ID NO: 28368 - DNA, 28 bp, synthetic construct
  source 1..28: mol_type = other DNA
agacagcacaaagggaactcccccatgg

SEQ ID NO: 28369 - DNA, 28 bp, synthetic construct
  source 1..28: mol_type = other DNA
gggaactcccccatggagcttcagatgg

SEQ ID NO: 28370 - DNA, 28 bp, synthetic construct
  source 1..28: mol_type = other DNA
agggctaccatctgaagctccatggggg

SEQ ID NO: 28371 - DNA, 28 bp, synthetic construct
  source 1..28: mol_type = other DNA
cagggctaccatctgaagctccatgggg

SEQ ID NO: 28372 - DNA, 28 bp, synthetic construct
  source 1..28: mol_type = other DNA
gcagggctaccatctgaagctccatggg

SEQ ID NO: 28373 - DNA, 28 bp, synthetic construct
  source 1..28: mol_type = other DNA
tgcagggctaccatctgaagctccatgg

SEQ ID NO: 28374 - DNA, 28 bp, synthetic construct
  source 1..28: mol_type = other DNA
tggcgtgaataattaagtgagtgcaggg

SEQ ID NO: 28375 - DNA, 28 bp, synthetic construct
  source 1..28: mol_type = other DNA
ctggcgtgaataattaagtgagtgcagg

SEQ ID NO: 28376 - DNA, 28 bp, synthetic construct
  source 1..28: mol_type = other DNA
gagggatgtcaggcagatttcatgctgg

SEQ ID NO: 28377 - DNA, 28 bp, synthetic construct
  source 1..28: mol_type = other DNA
caagaggatgaggaagagggatgtcagg

SEQ ID NO: 28378 - DNA, 28 bp, synthetic construct
  source 1..28: mol_type = other DNA
gttgctgtcaagaggatgaggaagaggg

SEQ ID NO: 28379 - DNA, 28 bp, synthetic construct
  source 1..28: mol_type = other DNA
tgttgctgtcaagaggatgaggaagagg

SEQ ID NO: 28380 - DNA, 28 bp, synthetic construct
  source 1..28: mol_type = other DNA
taatgctgttgctgtcaagaggatgagg

SEQ ID NO: 28381 - DNA, 28 bp, synthetic construct
  source 1..28: mol_type = other DNA
atcctcttgacagcaacagcattaaagg

SEQ ID NO: 28382 - DNA, 28 bp, synthetic construct
  source 1..28: mol_type = other DNA
atcctttaatgctgttgctgtcaagagg

SEQ ID NO: 28383 - DNA, 28 bp, synthetic construct
  source 1..28: mol_type = other DNA
cagcattaaaggattaagtagtatttgg

SEQ ID NO: 28384 - DNA, 28 bp, synthetic construct
  source 1..28: mol_type = other DNA
agcattaaaggattaagtagtatttggg

SEQ ID NO: 28385 - DNA, 28 bp, synthetic construct
  source 1..28: mol_type = other DNA
gcattaaaggattaagtagtatttgggg

SEQ ID NO: 28386 - DNA, 28 bp, synthetic construct
  source 1..28: mol_type = other DNA
gattaagtagtatttggggctctgaagg

SEQ ID NO: 28387 - DNA, 28 bp, synthetic construct
  source 1..28: mol_type = other DNA
attaagtagtatttggggctctgaaggg

SEQ ID NO: 28388 - DNA, 28 bp, synthetic construct
  source 1..28: mol_type = other DNA
ttaagtagtatttggggctctgaagggg

SEQ ID NO: 28389 - DNA, 28 bp, synthetic construct
  source 1..28: mol_type = other DNA
ggcctgaagagtgtttgtgtacaaaagg

SEQ ID NO: 28390 - DNA, 28 bp, synthetic construct
  source 1..28: mol_type = other DNA
ttccttttgtacacaaacactcttcagg

SEQ ID NO: 28391 - DNA, 28 bp, synthetic construct
  source 1..28: mol_type = other DNA
ctcacaatccaagtacataagacagcgg

SEQ ID NO: 28392 - DNA, 28 bp, synthetic construct
  source 1..28: mol_type = other DNA
agtgatgtccgctgtcttatgtacttgg

SEQ ID NO: 28393 - DNA, 28 bp, synthetic construct
  source 1..28: mol_type = other DNA
agtacataagacagcggacatcacttgg

SEQ ID NO: 28394 - DNA, 28 bp, synthetic construct
  source 1..28: mol_type = other DNA
gtacataagacagcggacatcacttggg

SEQ ID NO: 28395 - DNA, 28 bp, synthetic construct
  source 1..28: mol_type = other DNA
gtttacattgacctcctctgtatctagg

SEQ ID NO: 28396 - DNA, 28 bp, synthetic construct
  source 1..28: mol_type = other DNA
attgacctcctctgtatctaggcaatgg

SEQ ID NO: 28397 - DNA, 28 bp, synthetic construct
  source 1..28: mol_type = other DNA
agagaccattgcctagatacagaggagg

SEQ ID NO: 28398 - DNA, 28 bp, synthetic construct
  source 1..28: mol_type = other DNA
tgaagagaccattgcctagatacagagg

SEQ ID NO: 28399 - DNA, 28 bp, synthetic construct
  source 1..28: mol_type = other DNA
tcaaaatcaagcaccacacccccaatgg

SEQ ID NO: 28400 - DNA, 28 bp, synthetic construct
  source 1..28: mol_type = other DNA
tggagaactgcagccattgggggtgtgg

SEQ ID NO: 28401 - DNA, 28 bp, synthetic construct
  source 1..28: mol_type = other DNA
caggatggagaactgcagccattggggg

SEQ ID NO: 28402 - DNA, 28 bp, synthetic construct
  source 1..28: mol_type = other DNA
ccccaatggctgcagttctccatcctgg

SEQ ID NO: 28403 - DNA, 28 bp, synthetic construct
  source 1..28: mol_type = other DNA
accaggatggagaactgcagccattggg

SEQ ID NO: 28404 - DNA, 28 bp, synthetic construct
  source 1..28: mol_type = other DNA
aaccaggatggagaactgcagccattgg

SEQ ID NO: 28405 - DNA, 28 bp, synthetic construct
  source 1..28: mol_type = other DNA
tggctgcagttctccatcctggttaagg

SEQ ID NO: 28406 - DNA, 28 bp, synthetic construct
  source 1..28: mol_type = other DNA
tcagaaggagaggccttaaccaggatgg

SEQ ID NO: 28407 - DNA, 28 bp, synthetic construct
  source 1..28: mol_type = other DNA
atcctggttaaggcctctccttctgagg

SEQ ID NO: 28408 - DNA, 28 bp, synthetic construct
  source 1..28: mol_type = other DNA
ttcctcagaaggagaggccttaaccagg

SEQ ID NO: 28409 - DNA, 28 bp, synthetic construct
  source 1..28: mol_type = other DNA
ggaagaagtcattcctcagaaggagagg

SEQ ID NO: 28410 - DNA, 28 bp, synthetic construct
  source 1..28: mol_type = other DNA
taaatggaagaagtcattcctcagaagg

SEQ ID NO: 28411 - DNA, 28 bp, synthetic construct
  source 1..28: mol_type = other DNA
cctcagggttagactgactgttaaatgg

SEQ ID NO: 28412 - DNA, 28 bp, synthetic construct
  source 1..28: mol_type = other DNA
catttaacagtcagtctaaccctgaggg

SEQ ID NO: 28413 - DNA, 28 bp, synthetic construct
  source 1..28: mol_type = other DNA
taacagtcagtctaaccctgagggctgg

SEQ ID NO: 28414 - DNA, 28 bp, synthetic construct
  source 1..28: mol_type = other DNA
gtcagtctaaccctgagggctggagagg

SEQ ID NO: 28415 - DNA, 28 bp, synthetic construct
  source 1..28: mol_type = other DNA
tcagtctaaccctgagggctggagaggg

SEQ ID NO: 28416 - DNA, 28 bp, synthetic construct
  source 1..28: mol_type = other DNA
cctctgtggccctctccagccctcaggg

SEQ ID NO: 28417 - DNA, 28 bp, synthetic construct
  source 1..28: mol_type = other DNA
acctctgtggccctctccagccctcagg

SEQ ID NO: 28418 - DNA, 28 bp, synthetic construct
  source 1..28: mol_type = other DNA
gtagaggttgtgttaatgacctctgtgg

SEQ ID NO: 28419 - DNA, 28 bp, synthetic construct
  source 1..28: mol_type = other DNA
caacctctacacctgctgaacagtgtgg

SEQ ID NO: 28420 - DNA, 28 bp, synthetic construct
  source 1..28: mol_type = other DNA
ctgccacactgttcagcaggtgtagagg

SEQ ID NO: 28421 - DNA, 28 bp, synthetic construct
  source 1..28: mol_type = other DNA
ctctacacctgctgaacagtgtggcagg

SEQ ID NO: 28422 - DNA, 28 bp, synthetic construct
  source 1..28: mol_type = other DNA
tgttcttcctgccacactgttcagcagg

SEQ ID NO: 28423 - DNA, 28 bp, synthetic construct
  source 1..28: mol_type = other DNA
ctgaacagtgtggcaggaagaacatagg

SEQ ID NO: 28424 - DNA, 28 bp, synthetic construct
  source 1..28: mol_type = other DNA
tgaacagtgtggcaggaagaacataggg

SEQ ID NO: 28425 - DNA, 28 bp, synthetic construct
  source 1..28: mol_type = other DNA
gtgtggcaggaagaacatagggctgtgg

SEQ ID NO: 28426 - DNA, 28 bp, synthetic construct
  source 1..28: mol_type = other DNA
agacctaataacccaagagctaccttgg

SEQ ID NO: 28427 - DNA, 28 bp, synthetic construct
  source 1..28: mol_type = other DNA
tggccaaggtagctcttgggttattagg

SEQ ID NO: 28428 - DNA, 28 bp, synthetic construct
  source 1..28: mol_type = other DNA
ttggtcagtggccaaggtagctcttggg

SEQ ID NO: 28429 - DNA, 28 bp, synthetic construct
  source 1..28: mol_type = other DNA
cttggtcagtggccaaggtagctcttgg

SEQ ID NO: 28430 - DNA, 28 bp, synthetic construct
  source 1..28: mol_type = other DNA
agagctaccttggccactgaccaagtgg

SEQ ID NO: 28431 - DNA, 28 bp, synthetic construct
  source 1..28: mol_type = other DNA
gagctaccttggccactgaccaagtggg

SEQ ID NO: 28432 - DNA, 28 bp, synthetic construct
  source 1..28: mol_type = other DNA
agctaccttggccactgaccaagtgggg

SEQ ID NO: 28433 - DNA, 28 bp, synthetic construct
  source 1..28: mol_type = other DNA
gctaccttggccactgaccaagtggggg

SEQ ID NO: 28434 - DNA, 28 bp, synthetic construct
  source 1..28: mol_type = other DNA
ggtgcccccacttggtcagtggccaagg

SEQ ID NO: 28435 - DNA, 28 bp, synthetic construct
  source 1..28: mol_type = other DNA
ggccactgaccaagtgggggcaccttgg

SEQ ID NO: 28436 - DNA, 28 bp, synthetic construct
  source 1..28: mol_type = other DNA
gccactgaccaagtgggggcaccttggg

SEQ ID NO: 28437 - DNA, 28 bp, synthetic construct
  source 1..28: mol_type = other DNA
tcccaaggtgcccccacttggtcagtgg

SEQ ID NO: 28438 - DNA, 28 bp, synthetic construct
  source 1..28: mol_type = other DNA
gtaactttcccaaggtgcccccacttgg

SEQ ID NO: 28439 - DNA, 28 bp, synthetic construct
  source 1..28: mol_type = other DNA
agtctcagaggatgtaactttcccaagg

SEQ ID NO: 28440 - DNA, 28 bp, synthetic construct
  source 1..28: mol_type = other DNA
tgtggatgagaaaacagagtctcagagg

SEQ ID NO: 28441 - DNA, 28 bp, synthetic construct
  source 1..28: mol_type = other DNA
tctgagactctgttttctcatccacagg

SEQ ID NO: 28442 - DNA, 28 bp, synthetic construct
  source 1..28: mol_type = other DNA
actctgttttctcatccacaggatgagg

SEQ ID NO: 28443 - DNA, 28 bp, synthetic construct
  source 1..28: mol_type = other DNA
catctaatgcaacttcctcatcctgtgg

SEQ ID NO: 28444 - DNA, 28 bp, synthetic construct
  source 1..28: mol_type = other DNA
cacaggatgaggaagttgcattagatgg

SEQ ID NO: 28445 - DNA, 28 bp, synthetic construct
  source 1..28: mol_type = other DNA
gatggattttctgtgtcatcttgcttgg

SEQ ID NO: 28446 - DNA, 28 bp, synthetic construct
  source 1..28: mol_type = other DNA
atggattttctgtgtcatcttgcttggg

SEQ ID NO: 28447 - DNA, 28 bp, synthetic construct
  source 1..28: mol_type = other DNA
tttctgtgtcatcttgcttgggccatgg

SEQ ID NO: 28448 - DNA, 28 bp, synthetic construct
  source 1..28: mol_type = other DNA
ttctgtgtcatcttgcttgggccatggg

SEQ ID NO: 28449 - DNA, 28 bp, synthetic construct
  source 1..28: mol_type = other DNA
tctgtgtcatcttgcttgggccatgggg

SEQ ID NO: 28450 - DNA, 28 bp, synthetic construct
  source 1..28: mol_type = other DNA
gtttgactaaatgtgtggcaccccatgg

SEQ ID NO: 28451 - DNA, 28 bp, synthetic construct
  source 1..28: mol_type = other DNA
ccacacatttagtcaaacattattctgg

SEQ ID NO: 28452 - DNA, 28 bp, synthetic construct
  source 1..28: mol_type = other DNA
agtcaaacattattctggctgtttctgg

SEQ ID NO: 28453 - DNA, 28 bp, synthetic construct
  source 1..28: mol_type = other DNA
agtaacatttcaatctgagtaaagcagg

SEQ ID NO: 28454 - DNA, 28 bp, synthetic construct
  source 1..28: mol_type = other DNA
gtaaagcaggttgccctccctaacatgg

SEQ ID NO: 28455 - DNA, 28 bp, synthetic construct
  source 1..28: mol_type = other DNA
taaagcaggttgccctccctaacatggg

SEQ ID NO: 28456 - DNA, 28 bp, synthetic construct
  source 1..28: mol_type = other DNA
gcaggttgccctccctaacatgggtagg

SEQ ID NO: 28457 - DNA, 28 bp, synthetic construct
  source 1..28: mol_type = other DNA
gtctggggcctacccatgttagggaggg

SEQ ID NO: 28458 - DNA, 28 bp, synthetic construct
  source 1..28: mol_type = other DNA
tgtctggggcctacccatgttagggagg

SEQ ID NO: 28459 - DNA, 28 bp, synthetic construct
  source 1..28: mol_type = other DNA
aattgtctggggcctacccatgttaggg

SEQ ID NO: 28460 - DNA, 28 bp, synthetic construct
  source 1..28: mol_type = other DNA
caattgtctggggcctacccatgttagg

SEQ ID NO: 28461 - DNA, 28 bp, synthetic construct
  source 1..28: mol_type = other DNA
ctaacatgggtaggccccagacaattgg

SEQ ID NO: 28462 - DNA, 28 bp, synthetic construct
  source 1..28: mol_type = other DNA
gttctggctttcagccaattgtctgggg

SEQ ID NO: 28463 - DNA, 28 bp, synthetic construct
  source 1..28: mol_type = other DNA
tgttctggctttcagccaattgtctggg

SEQ ID NO: 28464 - DNA, 28 bp, synthetic construct
  source 1..28: mol_type = other DNA
ctgttctggctttcagccaattgtctgg

SEQ ID NO: 28465 - DNA, 28 bp, synthetic construct
  source 1..28: mol_type = other DNA
ggctgaaagccagaacagaatcaaaagg

SEQ ID NO: 28466 - DNA, 28 bp, synthetic construct
  source 1..28: mol_type = other DNA
aggggtctgccttttgattctgttctgg

SEQ ID NO: 28467 - DNA, 28 bp, synthetic construct
  source 1..28: mol_type = other DNA
aaaaggcagacccctcctagatataagg

SEQ ID NO: 28468 - DNA, 28 bp, synthetic construct
  source 1..28: mol_type = other DNA
aaaggcagacccctcctagatataaggg

SEQ ID NO: 28469 - DNA, 28 bp, synthetic construct
  source 1..28: mol_type = other DNA
aaggcagacccctcctagatataagggg

SEQ ID NO: 28470 - DNA, 28 bp, synthetic construct
  source 1..28: mol_type = other DNA
aggcagacccctcctagatataaggggg

SEQ ID NO: 28471 - DNA, 28 bp, synthetic construct
  source 1..28: mol_type = other DNA
agagattcccccttatatctaggagggg

SEQ ID NO: 28472 - DNA, 28 bp, synthetic construct
  source 1..28: mol_type = other DNA
aagagattcccccttatatctaggaggg

SEQ ID NO: 28473 - DNA, 28 bp, synthetic construct
  source 1..28: mol_type = other DNA
aaagagattcccccttatatctaggagg

SEQ ID NO: 28474 - DNA, 28 bp, synthetic construct
  source 1..28: mol_type = other DNA
cagaaagagattcccccttatatctagg

SEQ ID NO: 28475 - DNA, 28 bp, synthetic construct
  source 1..28: mol_type = other DNA
gggaaaaactgatgtcgcaggctcaagg

SEQ ID NO: 28476 - DNA, 28 bp, synthetic construct
  source 1..28: mol_type = other DNA
aaaggcagggaaaaactgatgtcgcagg

SEQ ID NO: 28477 - DNA, 28 bp, synthetic construct
  source 1..28: mol_type = other DNA
tgcgacatcagtttttccctgcctttgg

SEQ ID NO: 28478 - DNA, 28 bp, synthetic construct
  source 1..28: mol_type = other DNA
gtgtttcattttgagtccaaaggcaggg

SEQ ID NO: 28479 - DNA, 28 bp, synthetic construct
  source 1..28: mol_type = other DNA
agtgtttcattttgagtccaaaggcagg

SEQ ID NO: 28480 - DNA, 28 bp, synthetic construct
  source 1..28: mol_type = other DNA
tgcctttggactcaaaatgaaacactgg

SEQ ID NO: 28481 - DNA, 28 bp, synthetic construct
  source 1..28: mol_type = other DNA
gcctttggactcaaaatgaaacactggg

SEQ ID NO: 28482 - DNA, 28 bp, synthetic construct
  source 1..28: mol_type = other DNA
acccagtgtttcattttgagtccaaagg

SEQ ID NO: 28483 - DNA, 28 bp, synthetic construct
  source 1..28: mol_type = other DNA
tcaaaatgaaacactgggttttcctagg

SEQ ID NO: 28484 - DNA, 28 bp, synthetic construct
  source 1..28: mol_type = other DNA
tcaaaggctggcagacttaagacctagg

SEQ ID NO: 28485 - DNA, 28 bp, synthetic construct
  source 1..28: mol_type = other DNA
gtcttaagtctgccagcctttgaactgg

SEQ ID NO: 28486 - DNA, 28 bp, synthetic construct
  source 1..28: mol_type = other DNA
gtggtgtgagttccagttcaaaggctgg

SEQ ID NO: 28487 - DNA, 28 bp, synthetic construct
  source 1..28: mol_type = other DNA
gcctttgaactggaactcacaccactgg

SEQ ID NO: 28488 - DNA, 28 bp, synthetic construct
  source 1..28: mol_type = other DNA
gccagtggtgtgagttccagttcaaagg

SEQ ID NO: 28489 - DNA, 28 bp, synthetic construct
  source 1..28: mol_type = other DNA
catgctggagatgcaggagagccagtgg

SEQ ID NO: 28490 - DNA, 28 bp, synthetic construct
  source 1..28: mol_type = other DNA
gaatgactcagcatgctggagatgcagg

SEQ ID NO: 28491 - DNA, 28 bp, synthetic construct
  source 1..28: mol_type = other DNA
agatctgcagaatgactcagcatgctgg

SEQ ID NO: 28492 - DNA, 28 bp, synthetic construct
  source 1..28: mol_type = other DNA
gcatgctgagtcattctgcagatcttgg

SEQ ID NO: 28493 - DNA, 28 bp, synthetic construct
  source 1..28: mol_type = other DNA
aaggaattggcttatgtgattatggagg

SEQ ID NO: 28494 - DNA, 28 bp, synthetic construct
  source 1..28: mol_type = other DNA
gataaggaattggcttatgtgattatgg

SEQ ID NO: 28495 - DNA, 28 bp, synthetic construct
  source 1..28: mol_type = other DNA
tcacataagccaattccttatcctaagg

SEQ ID NO: 28496 - DNA, 28 bp, synthetic construct
  source 1..28: mol_type = other DNA
cacgtaaatccttaggataaggaattgg

SEQ ID NO: 28497 - DNA, 28 bp, synthetic construct
  source 1..28: mol_type = other DNA
acaatacacgtaaatccttaggataagg

SEQ ID NO: 28498 - DNA, 28 bp, synthetic construct
  source 1..28: mol_type = other DNA
tggaaaacaatacacgtaaatccttagg

SEQ ID NO: 28499 - DNA, 28 bp, synthetic construct
  source 1..28: mol_type = other DNA
gtgtattgttttccatccatcctattgg

SEQ ID NO: 28500 - DNA, 28 bp, synthetic construct
  source 1..28: mol_type = other DNA
agggaaatagaaccaataggatggatgg

SEQ ID NO: 28501 - DNA, 28 bp, synthetic construct
  source 1..28: mol_type = other DNA
atccatcctattggttctatttccctgg

SEQ ID NO: 28502 - DNA, 28 bp, synthetic construct
  source 1..28: mol_type = other DNA
ttccagggaaatagaaccaataggatgg

SEQ ID NO: 28503 - DNA, 28 bp, synthetic construct
  source 1..28: mol_type = other DNA
gattttccagggaaatagaaccaatagg

SEQ ID NO: 28504 - DNA, 28 bp, synthetic construct
  source 1..28: mol_type = other DNA
ttggggattgtattaggattttccaggg

SEQ ID NO: 28505 - DNA, 28 bp, synthetic construct
  source 1..28: mol_type = other DNA
tttggggattgtattaggattttccagg

SEQ ID NO: 28506 - DNA, 28 bp, synthetic construct
  source 1..28: mol_type = other DNA
aaagttcatctttggggattgtattagg

SEQ ID NO: 28507 - DNA, 28 bp, synthetic construct
  source 1..28: mol_type = other DNA
ggttagaaatgaaagttcatctttgggg

SEQ ID NO: 28508 - DNA, 28 bp, synthetic construct
  source 1..28: mol_type = other DNA
gggttagaaatgaaagttcatctttggg

SEQ ID NO: 28509 - DNA, 28 bp, synthetic construct
  source 1..28: mol_type = other DNA
ggggttagaaatgaaagttcatctttgg

SEQ ID NO: 28510 - DNA, 28 bp, synthetic construct
  source 1..28: mol_type = other DNA
actttcatttctaacccctaccaaatgg

SEQ ID NO: 28511 - DNA, 28 bp, synthetic construct
  source 1..28: mol_type = other DNA
agtggatcagatggccatttggtagggg

SEQ ID NO: 28512 - DNA, 28 bp, synthetic construct
  source 1..28: mol_type = other DNA
aagtggatcagatggccatttggtaggg

SEQ ID NO: 28513 - DNA, 28 bp, synthetic construct
  source 1..28: mol_type = other DNA
caagtggatcagatggccatttggtagg

SEQ ID NO: 28514 - DNA, 28 bp, synthetic construct
  source 1..28: mol_type = other DNA
tgtacaagtggatcagatggccatttgg

SEQ ID NO: 28515 - DNA, 28 bp, synthetic construct
  source 1..28: mol_type = other DNA
ctaagaggtgtacaagtggatcagatgg

SEQ ID NO: 28516 - DNA, 28 bp, synthetic construct
  source 1..28: mol_type = other DNA
gtcttgtctctaagaggtgtacaagtgg

SEQ ID NO: 28517 - DNA, 28 bp, synthetic construct
  source 1..28: mol_type = other DNA
ggagcagtgcagtcttgtctctaagagg

SEQ ID NO: 28518 - DNA, 28 bp, synthetic construct
  source 1..28: mol_type = other DNA
agagacaagactgcactgctccctgtgg

SEQ ID NO: 28519 - DNA, 28 bp, synthetic construct
  source 1..28: mol_type = other DNA
ccctgtggcacctcaccctgctctaagg

SEQ ID NO: 28520 - DNA, 28 bp, synthetic construct
  source 1..28: mol_type = other DNA
cccttagagcagggtgaggtgccacagg

SEQ ID NO: 28521 - DNA, 28 bp, synthetic construct
  source 1..28: mol_type = other DNA
gcacctcaccctgctctaagggcagtgg

SEQ ID NO: 28522 - DNA, 28 bp, synthetic construct
  source 1..28: mol_type = other DNA
cctcaccctgctctaagggcagtggagg

SEQ ID NO: 28523 - DNA, 28 bp, synthetic construct
  source 1..28: mol_type = other DNA
gctgacctccactgcccttagagcaggg

SEQ ID NO: 28524 - DNA, 28 bp, synthetic construct
  source 1..28: mol_type = other DNA
ggctgacctccactgcccttagagcagg

SEQ ID NO: 28525 - DNA, 28 bp, synthetic construct
  source 1..28: mol_type = other DNA
ctaagggcagtggaggtcagcctcttgg

SEQ ID NO: 28526 - DNA, 28 bp, synthetic construct
  source 1..28: mol_type = other DNA
taagggcagtggaggtcagcctcttggg

SEQ ID NO: 28527 - DNA, 28 bp, synthetic construct
  source 1..28: mol_type = other DNA
tcagcctcttgggaagcactaccccagg

SEQ ID NO: 28528 - DNA, 28 bp, synthetic construct
  source 1..28: mol_type = other DNA
gtcacctggggtagtgcttcccaagagg

SEQ ID NO: 28529 - DNA, 28 bp, synthetic construct
  source 1..28: mol_type = other DNA
gctggttcagctttggagtcacctgggg

SEQ ID NO: 28530 - DNA, 28 bp, synthetic construct
  source 1..28: mol_type = other DNA
ggctggttcagctttggagtcacctggg

SEQ ID NO: 28531 - DNA, 28 bp, synthetic construct
  source 1..28: mol_type = other DNA
tggctggttcagctttggagtcacctgg

SEQ ID NO: 28532 - DNA, 28 bp, synthetic construct
  source 1..28: mol_type = other DNA
ggtgggaatgtggctggttcagctttgg

SEQ ID NO: 28533 - DNA, 28 bp, synthetic construct
  source 1..28: mol_type = other DNA
cactctttgtgggtgggaatgtggctgg

SEQ ID NO: 28534 - DNA, 28 bp, synthetic construct
  source 1..28: mol_type = other DNA
gaaacactctttgtgggtgggaatgtgg

SEQ ID NO: 28535 - DNA, 28 bp, synthetic construct
  source 1..28: mol_type = other DNA
tgttggagaaacactctttgtgggtggg

SEQ ID NO: 28536 - DNA, 28 bp, synthetic construct
  source 1..28: mol_type = other DNA
ctgttggagaaacactctttgtgggtgg

SEQ ID NO: 28537 - DNA, 28 bp, synthetic construct
  source 1..28: mol_type = other DNA
cacccacaaagagtgtttctccaacagg

SEQ ID NO: 28538 - DNA, 28 bp, synthetic construct
  source 1..28: mol_type = other DNA
cacctgttggagaaacactctttgtggg

SEQ ID NO: 28539 - DNA, 28 bp, synthetic construct
  source 1..28: mol_type = other DNA
acacctgttggagaaacactctttgtgg

SEQ ID NO: 28540 - DNA, 28 bp, synthetic construct
  source 1..28: mol_type = other DNA
tctgctcaggtcaaatcacacctgttgg

SEQ ID NO: 28541 - DNA, 28 bp, synthetic construct
  source 1..28: mol_type = other DNA
gataaaatttctactgtatctgctcagg

SEQ ID NO: 28542 - DNA, 28 bp, synthetic construct
  source 1..28: mol_type = other DNA
cattgacataattacagtgaaagcaggg

SEQ ID NO: 28543 - DNA, 28 bp, synthetic construct
  source 1..28: mol_type = other DNA
acattgacataattacagtgaaagcagg

SEQ ID NO: 28544 - DNA, 28 bp, synthetic construct
  source 1..28: mol_type = other DNA
gctttcactgtaattatgtcaatgtagg

SEQ ID NO: 28545 - DNA, 28 bp, synthetic construct
  source 1..28: mol_type = other DNA
atgtcaatgtaggctgagattgccttgg

SEQ ID NO: 28546 - DNA, 28 bp, synthetic construct
  source 1..28: mol_type = other DNA
ctgagattgccttggttgttattgttgg

SEQ ID NO: 28547 - DNA, 28 bp, synthetic construct
  source 1..28: mol_type = other DNA
tgagattgccttggttgttattgttggg

SEQ ID NO: 28548 - DNA, 28 bp, synthetic construct
  source 1..28: mol_type = other DNA
agataaaacccaacaataacaaccaagg

SEQ ID NO: 28549 - DNA, 28 bp, synthetic construct
  source 1..28: mol_type = other DNA
gttattgttgggttttatctcgttttgg

SEQ ID NO: 28550 - DNA, 28 bp, synthetic construct
  source 1..28: mol_type = other DNA
ttattgttgggttttatctcgttttggg

SEQ ID NO: 28551 - DNA, 28 bp, synthetic construct
  source 1..28: mol_type = other DNA
gggttttatctcgttttgggtttcctgg

SEQ ID NO: 28552 - DNA, 28 bp, synthetic construct
  source 1..28: mol_type = other DNA
ttcctggttatcacatactgttcgttgg

SEQ ID NO: 28553 - DNA, 28 bp, synthetic construct
  source 1..28: mol_type = other DNA
agccaacgaacagtatgtgataaccagg

SEQ ID NO: 28554 - DNA, 28 bp, synthetic construct
  source 1..28: mol_type = other DNA
tgaaatggatgtgaaaatgagttaaggg

SEQ ID NO: 28555 - DNA, 28 bp, synthetic construct
  source 1..28: mol_type = other DNA
gtgaaatggatgtgaaaatgagttaagg

SEQ ID NO: 28556 - DNA, 28 bp, synthetic construct
  source 1..28: mol_type = other DNA
taactcattttcacatccatttcactgg

SEQ ID NO: 28557 - DNA, 28 bp, synthetic construct
  source 1..28: mol_type = other DNA
aactcattttcacatccatttcactggg

SEQ ID NO: 28558 - DNA, 28 bp, synthetic construct
  source 1..28: mol_type = other DNA
attttcacatccatttcactgggtgtgg

SEQ ID NO: 28559 - DNA, 28 bp, synthetic construct
  source 1..28: mol_type = other DNA
ggtgatttggccacacccagtgaaatgg

SEQ ID NO: 28560 - DNA, 28 bp, synthetic construct
  source 1..28: mol_type = other DNA
ctttcagaagtgtcaggtggtgatttgg

SEQ ID NO: 28561 - DNA, 28 bp, synthetic construct
  source 1..28: mol_type = other DNA
aaaagtctctttcagaagtgtcaggtgg

SEQ ID NO: 28562 - DNA, 28 bp, synthetic construct
  source 1..28: mol_type = other DNA
actaaaagtctctttcagaagtgtcagg

SEQ ID NO: 28563 - DNA, 28 bp, synthetic construct
  source 1..28: mol_type = other DNA
cttctgaaagagacttttagtacatagg

SEQ ID NO: 28564 - DNA, 28 bp, synthetic construct
  source 1..28: mol_type = other DNA
ttctgaaagagacttttagtacataggg

SEQ ID NO: 28565 - DNA, 28 bp, synthetic construct
  source 1..28: mol_type = other DNA
gaaagagacttttagtacatagggaagg

SEQ ID NO: 28566 - DNA, 28 bp, synthetic construct
  source 1..28: mol_type = other DNA
gatgttggtatagtaaaaaatataaagg

SEQ ID NO: 28567 - DNA, 28 bp, synthetic construct
  source 1..28: mol_type = other DNA
tataccaacatcatcttgttaccttagg

SEQ ID NO: 28568 - DNA, 28 bp, synthetic construct
  source 1..28: mol_type = other DNA
ataccaacatcatcttgttaccttaggg

SEQ ID NO: 28569 - DNA, 28 bp, synthetic construct
  source 1..28: mol_type = other DNA
tggccctaaggtaacaagatgatgttgg

SEQ ID NO: 28570 - DNA, 28 bp, synthetic construct
  source 1..28: mol_type = other DNA
aagaactgcaaaaattctggccctaagg

SEQ ID NO: 28571 - DNA, 28 bp, synthetic construct
  source 1..28: mol_type = other DNA
gacagggtaagaactgcaaaaattctgg

SEQ ID NO: 28572 - DNA, 28 bp, synthetic construct
  source 1..28: mol_type = other DNA
ggtggacatggttctttagatgacaggg

SEQ ID NO: 28573 - DNA, 28 bp, synthetic construct
  source 1..28: mol_type = other DNA
aggtggacatggttctttagatgacagg

SEQ ID NO: 28574 - DNA, 28 bp, synthetic construct
  source 1..28: mol_type = other DNA
gatgacacagagggagaggtggacatgg

SEQ ID NO: 28575 - DNA, 28 bp, synthetic construct
  source 1..28: mol_type = other DNA
tctctggatgacacagagggagaggtgg

SEQ ID NO: 28576 - DNA, 28 bp, synthetic construct
  source 1..28: mol_type = other DNA
caatctctggatgacacagagggagagg

SEQ ID NO: 28577 - DNA, 28 bp, synthetic construct
  source 1..28: mol_type = other DNA
ctctccctctgtgtcatccagagattgg

SEQ ID NO: 28578 - DNA, 28 bp, synthetic construct
  source 1..28: mol_type = other DNA
caatccaatctctggatgacacagaggg

SEQ ID NO: 28579 - DNA, 28 bp, synthetic construct
  source 1..28: mol_type = other DNA
gcaatccaatctctggatgacacagagg

SEQ ID NO: 28580 - DNA, 28 bp, synthetic construct
  source 1..28: mol_type = other DNA
atgatgtactgtgcaatccaatctctgg

SEQ ID NO: 28581 - DNA, 28 bp, synthetic construct
  source 1..28: mol_type = other DNA
tgcacagtacatcattaaccctcatagg

SEQ ID NO: 28582 - DNA, 28 bp, synthetic construct
  source 1..28: mol_type = other DNA
tacatcattaaccctcataggaaacagg

SEQ ID NO: 28583 - DNA, 28 bp, synthetic construct
  source 1..28: mol_type = other DNA
attaaccctcataggaaacaggagatgg

SEQ ID NO: 28584 - DNA, 28 bp, synthetic construct
  source 1..28: mol_type = other DNA
gtgtgccatctcctgtttcctatgaggg

SEQ ID NO: 28585 - DNA, 28 bp, synthetic construct
  source 1..28: mol_type = other DNA
tgtgtgccatctcctgtttcctatgagg

SEQ ID NO: 28586 - DNA, 28 bp, synthetic construct
  source 1..28: mol_type = other DNA
agggtgctagtggggagtgcagcaaggg

SEQ ID NO: 28587 - DNA, 28 bp, synthetic construct
  source 1..28: mol_type = other DNA
gagggtgctagtggggagtgcagcaagg

SEQ ID NO: 28588 - DNA, 28 bp, synthetic construct
  source 1..28: mol_type = other DNA
cactccccactagcaccctccctcctgg

SEQ ID NO: 28589 - DNA, 28 bp, synthetic construct
  source 1..28: mol_type = other DNA
ctggccaggagggagggtgctagtgggg

SEQ ID NO: 28590 - DNA, 28 bp, synthetic construct
  source 1..28: mol_type = other DNA
actggccaggagggagggtgctagtggg

SEQ ID NO: 28591 - DNA, 28 bp, synthetic construct
  source 1..28: mol_type = other DNA
cactggccaggagggagggtgctagtgg

SEQ ID NO: 28592 - DNA, 28 bp, synthetic construct
  source 1..28: mol_type = other DNA
cactagcaccctccctcctggccagtgg

SEQ ID NO: 28593 - DNA, 28 bp, synthetic construct
  source 1..28: mol_type = other DNA
gctggagaccactggccaggagggaggg

SEQ ID NO: 28594 - DNA, 28 bp, synthetic construct
  source 1..28: mol_type = other DNA
agctggagaccactggccaggagggagg

SEQ ID NO: 28595 - DNA, 28 bp, synthetic construct
  source 1..28: mol_type = other DNA
cagagctggagaccactggccaggaggg

SEQ ID NO: 28596 - DNA, 28 bp, synthetic construct
  source 1..28: mol_type = other DNA
tcagagctggagaccactggccaggagg

SEQ ID NO: 28597 - DNA, 28 bp, synthetic construct
  source 1..28: mol_type = other DNA
aagtcagagctggagaccactggccagg

SEQ ID NO: 28598 - DNA, 28 bp, synthetic construct
  source 1..28: mol_type = other DNA
atgtgaagtcagagctggagaccactgg

SEQ ID NO: 28599 - DNA, 28 bp, synthetic construct
  source 1..28: mol_type = other DNA
ggtgattgtaatgtgaagtcagagctgg

SEQ ID NO: 28600 - DNA, 28 bp, synthetic construct
  source 1..28: mol_type = other DNA
ttttttttttttttttaagatttctagg

SEQ ID NO: 28601 - DNA, 28 bp, synthetic construct
  source 1..28: mol_type = other DNA
agaaaagaaaagaaagaaaaatgccagg

SEQ ID NO: 28602 - DNA, 28 bp, synthetic construct
  source 1..28: mol_type = other DNA
ctaaatcagaatcagaggttgagcctgg

SEQ ID NO: 28603 - DNA, 28 bp, synthetic construct
  source 1..28: mol_type = other DNA
gctcaacctctgattctgatttagttgg

SEQ ID NO: 28604 - DNA, 28 bp, synthetic construct
  source 1..28: mol_type = other DNA
caacctctgattctgatttagttggagg

SEQ ID NO: 28605 - DNA, 28 bp, synthetic construct
  source 1..28: mol_type = other DNA
aacctctgattctgatttagttggaggg

SEQ ID NO: 28606 - DNA, 28 bp, synthetic construct
  source 1..28: mol_type = other DNA
acctctgattctgatttagttggagggg

SEQ ID NO: 28607 - DNA, 28 bp, synthetic construct
  source 1..28: mol_type = other DNA
gcccctccaactaaatcagaatcagagg

SEQ ID NO: 28608 - DNA, 28 bp, synthetic construct
  source 1..28: mol_type = other DNA
gattctgatttagttggaggggctgagg

SEQ ID NO: 28609 - DNA, 28 bp, synthetic construct
  source 1..28: mol_type = other DNA
tctgatttagttggaggggctgaggagg

SEQ ID NO: 28610 - DNA, 28 bp, synthetic construct
  source 1..28: mol_type = other DNA
ggaggggctgaggaggaaagatgcttgg

SEQ ID NO: 28611 - DNA, 28 bp, synthetic construct
  source 1..28: mol_type = other DNA
gaggggctgaggaggaaagatgcttggg

SEQ ID NO: 28612 - DNA, 28 bp, synthetic construct
  source 1..28: mol_type = other DNA
gcttgggcattagtaagaatgctttagg

SEQ ID NO: 28613 - DNA, 28 bp, synthetic construct
  source 1..28: mol_type = other DNA
gctttaggtgattctaatgtacagcagg

SEQ ID NO: 28614 - DNA, 28 bp, synthetic construct
  source 1..28: mol_type = other DNA
caggctgagaaccagtgttctgtctagg

SEQ ID NO: 28615 - DNA, 28 bp, synthetic construct
  source 1..28: mol_type = other DNA
ctgatctctggcctagacagaacactgg

SEQ ID NO: 28616 - DNA, 28 bp, synthetic construct
  source 1..28: mol_type = other DNA
ttaacagacaaagtttgctgatctctgg

SEQ ID NO: 28617 - DNA, 28 bp, synthetic construct
  source 1..28: mol_type = other DNA
taaagagccagaaagcaaatattatagg

SEQ ID NO: 28618 - DNA, 28 bp, synthetic construct
  source 1..28: mol_type = other DNA
cgcaaagcctataatatttgctttctgg

SEQ ID NO: 28619 - DNA, 28 bp, synthetic construct
  source 1..28: mol_type = other DNA
cagaaagcaaatattataggctttgcgg

SEQ ID NO: 28620 - DNA, 28 bp, synthetic construct
  source 1..28: mol_type = other DNA
agaaagcaaatattataggctttgcggg

SEQ ID NO: 28621 - DNA, 28 bp, synthetic construct
  source 1..28: mol_type = other DNA
aatattataggctttgcgggccaaatgg

SEQ ID NO: 28622 - DNA, 28 bp, synthetic construct
  source 1..28: mol_type = other DNA
ctgagcagttgctttagagaccatttgg

SEQ ID NO: 28623 - DNA, 28 bp, synthetic construct
  source 1..28: mol_type = other DNA
ccttaaacaatacataataaacaaatgg

SEQ ID NO: 28624 - DNA, 28 bp, synthetic construct
  source 1..28: mol_type = other DNA
cttaaacaatacataataaacaaatggg

SEQ ID NO: 28625 - DNA, 28 bp, synthetic construct
  source 1..28: mol_type = other DNA
cttgtttttataaataaagttgtattgg

SEQ ID NO: 28626 - DNA, 28 bp, synthetic construct
  source 1..28: mol_type = other DNA
aactttatttataaaaacaagcaacagg

SEQ ID NO: 28627 - DNA, 28 bp, synthetic construct
  source 1..28: mol_type = other DNA
taatgaaatagcttctggggcaaaatgg

SEQ ID NO: 28628 - DNA, 28 bp, synthetic construct
  source 1..28: mol_type = other DNA
tgatcaactaatgaaatagcttctgggg

SEQ ID NO: 28629 - DNA, 28 bp, synthetic construct
  source 1..28: mol_type = other DNA
ttgatcaactaatgaaatagcttctggg

SEQ ID NO: 28630 - DNA, 28 bp, synthetic construct
  source 1..28: mol_type = other DNA
attgatcaactaatgaaatagcttctgg

SEQ ID NO: 28631 - DNA, 28 bp, synthetic construct
  source 1..28: mol_type = other DNA
tcatcacccagttttaaaatagttgtgg

SEQ ID NO: 28632 - DNA, 28 bp, synthetic construct
  source 1..28: mol_type = other DNA
catcacccagttttaaaatagttgtggg

SEQ ID NO: 28633 - DNA, 28 bp, synthetic construct
  source 1..28: mol_type = other DNA
ctgggcccacaactattttaaaactggg

SEQ ID NO: 28634 - DNA, 28 bp, synthetic construct
  source 1..28: mol_type = other DNA
gctgggcccacaactattttaaaactgg

SEQ ID NO: 28635 - DNA, 28 bp, synthetic construct
  source 1..28: mol_type = other DNA
taaaatagttgtgggcccagcacagtgg

SEQ ID NO: 28636 - DNA, 28 bp, synthetic construct
  source 1..28: mol_type = other DNA
gattacaggtgtgagccactgtgctggg

SEQ ID NO: 28637 - DNA, 28 bp, synthetic construct
  source 1..28: mol_type = other DNA
ggattacaggtgtgagccactgtgctgg

SEQ ID NO: 28638 - DNA, 28 bp, synthetic construct
  source 1..28: mol_type = other DNA
ccgactctgaaagctctgggattacagg

SEQ ID NO: 28639 - DNA, 28 bp, synthetic construct
  source 1..28: mol_type = other DNA
atcccagagctttcagagtcggagaagg

SEQ ID NO: 28640 - DNA, 28 bp, synthetic construct
  source 1..28: mol_type = other DNA
ttccttctccgactctgaaagctctggg

SEQ ID NO: 28641 - DNA, 28 bp, synthetic construct
  source 1..28: mol_type = other DNA
cttccttctccgactctgaaagctctgg

SEQ ID NO: 28642 - DNA, 28 bp, synthetic construct
  source 1..28: mol_type = other DNA
cagagctttcagagtcggagaaggaagg

SEQ ID NO: 28643 - DNA, 28 bp, synthetic construct
  source 1..28: mol_type = other DNA
gagtcggagaaggaaggactgcttgagg

SEQ ID NO: 28644 - DNA, 28 bp, synthetic construct
  source 1..28: mol_type = other DNA
ggagaaggaaggactgcttgaggccagg

SEQ ID NO: 28645 - DNA, 28 bp, synthetic construct
  source 1..28: mol_type = other DNA
aggactgcttgaggccaggagatcaagg

SEQ ID NO: 28646 - DNA, 28 bp, synthetic construct
  source 1..28: mol_type = other DNA
atagctcattgtaaccttgatctcctgg

SEQ ID NO: 28647 - DNA, 28 bp, synthetic construct
  source 1..28: mol_type = other DNA
tgagctatgatcatgcactccagcctgg

SEQ ID NO: 28648 - DNA, 28 bp, synthetic construct
  source 1..28: mol_type = other DNA
gagctatgatcatgcactccagcctggg

SEQ ID NO: 28649 - DNA, 28 bp, synthetic construct
  source 1..28: mol_type = other DNA
cagggtcttactctgttgcccaggctgg

SEQ ID NO: 28650 - DNA, 28 bp, synthetic construct
  source 1..28: mol_type = other DNA
gtgacagggtcttactctgttgcccagg

SEQ ID NO: 28651 - DNA, 28 bp, synthetic construct
  source 1..28: mol_type = other DNA
atttttttttttgttctaagtgacaggg

SEQ ID NO: 28652 - DNA, 28 bp, synthetic construct
  source 1..28: mol_type = other DNA
gatttttttttttgttctaagtgacagg

SEQ ID NO: 28653 - DNA, 28 bp, synthetic construct
  source 1..28: mol_type = other DNA
cacacacacacacacacacacacactgg

SEQ ID NO: 28654 - DNA, 28 bp, synthetic construct
  source 1..28: mol_type = other DNA
cacacacacacacacacactggttatgg

SEQ ID NO: 28655 - DNA, 28 bp, synthetic construct
  source 1..28: mol_type = other DNA
agagtctctggtgtcacagacaagatgg

SEQ ID NO: 28656 - DNA, 28 bp, synthetic construct
  source 1..28: mol_type = other DNA
tctgtgacaccagagactctcaaagtgg

SEQ ID NO: 28657 - DNA, 28 bp, synthetic construct
  source 1..28: mol_type = other DNA
tgacaccagagactctcaaagtggctgg

SEQ ID NO: 28658 - DNA, 28 bp, synthetic construct
  source 1..28: mol_type = other DNA
ttcagccagccactttgagagtctctgg

SEQ ID NO: 28659 - DNA, 28 bp, synthetic construct
  source 1..28: mol_type = other DNA
ctgaaatcaatattcactctctatccgg

SEQ ID NO: 28660 - DNA, 28 bp, synthetic construct
  source 1..28: mol_type = other DNA
ttcgtctgatacatgaagggaatgccgg

SEQ ID NO: 28661 - DNA, 28 bp, synthetic construct
  source 1..28: mol_type = other DNA
tgggatcattcgtctgatacatgaaggg

SEQ ID NO: 28662 - DNA, 28 bp, synthetic construct
  source 1..28: mol_type = other DNA
atgggatcattcgtctgatacatgaagg

SEQ ID NO: 28663 - DNA, 28 bp, synthetic construct
  source 1..28: mol_type = other DNA
gaacaagtctttttcttgtttagatggg

SEQ ID NO: 28664 - DNA, 28 bp, synthetic construct
  source 1..28: mol_type = other DNA
agaacaagtctttttcttgtttagatgg

SEQ ID NO: 28665 - DNA, 28 bp, synthetic construct
  source 1..28: mol_type = other DNA
aaacaagaaaaagacttgttcttagagg

SEQ ID NO: 28666 - DNA, 28 bp, synthetic construct
  source 1..28: mol_type = other DNA
cagcagtgagtaatgggagacagaaagg

SEQ ID NO: 28667 - DNA, 28 bp, synthetic construct
  source 1..28: mol_type = other DNA
atataataaggcagcagtgagtaatggg

SEQ ID NO: 28668 - DNA, 28 bp, synthetic construct
  source 1..28: mol_type = other DNA
catataataaggcagcagtgagtaatgg

SEQ ID NO: 28669 - DNA, 28 bp, synthetic construct
  source 1..28: mol_type = other DNA
agcagacgtttgtgaacatataataagg

SEQ ID NO: 28670 - DNA, 28 bp, synthetic construct
  source 1..28: mol_type = other DNA
atgggtgagcttaagtcagtttctgagg

SEQ ID NO: 28671 - DNA, 28 bp, synthetic construct
  source 1..28: mol_type = other DNA
aaagcatggtttggaaactacagatggg

SEQ ID NO: 28672 - DNA, 28 bp, synthetic construct
  source 1..28: mol_type = other DNA
gaaagcatggtttggaaactacagatgg

SEQ ID NO: 28673 - DNA, 28 bp, synthetic construct
  source 1..28: mol_type = other DNA
agctttcaagggggaaagcatggtttgg

SEQ ID NO: 28674 - DNA, 28 bp, synthetic construct
  source 1..28: mol_type = other DNA
aaaccatgctttcccccttgaaagctgg

SEQ ID NO: 28675 - DNA, 28 bp, synthetic construct
  source 1..28: mol_type = other DNA
aaccatgctttcccccttgaaagctggg

SEQ ID NO: 28676 - DNA, 28 bp, synthetic construct
  source 1..28: mol_type = other DNA
gtcccagctttcaagggggaaagcatgg

SEQ ID NO: 28677 - DNA, 28 bp, synthetic construct
  source 1..28: mol_type = other DNA
gacaaacatgtcccagctttcaaggggg

SEQ ID NO: 28678 - DNA, 28 bp, synthetic construct
  source 1..28: mol_type = other DNA
tgacaaacatgtcccagctttcaagggg

SEQ ID NO: 28679 - DNA, 28 bp, synthetic construct
  source 1..28: mol_type = other DNA
ttgacaaacatgtcccagctttcaaggg

SEQ ID NO: 28680 - DNA, 28 bp, synthetic construct
  source 1..28: mol_type = other DNA
tttgacaaacatgtcccagctttcaagg

SEQ ID NO: 28681 - DNA, 28 bp, synthetic construct
  source 1..28: mol_type = other DNA
tttgtcaaaatcatttacaatcttctgg

SEQ ID NO: 28682 - DNA, 28 bp, synthetic construct
  source 1..28: mol_type = other DNA
taatattttgtgaatcaaggagaatagg

SEQ ID NO: 28683 - DNA, 28 bp, synthetic construct
  source 1..28: mol_type = other DNA
actttagataatattttgtgaatcaagg

SEQ ID NO: 28684 - DNA, 28 bp, synthetic construct
  source 1..28: mol_type = other DNA
ttgattcacaaaatattatctaaagtgg

SEQ ID NO: 28685 - DNA, 28 bp, synthetic construct
  source 1..28: mol_type = other DNA
cggaaggaacttgcagatgtgattgtgg

SEQ ID NO: 28686 - DNA, 28 bp, synthetic construct
  source 1..28: mol_type = other DNA
acatctgcaagttccttccgtgcccagg

SEQ ID NO: 28687 - DNA, 28 bp, synthetic construct
  source 1..28: mol_type = other DNA
tctgcaagttccttccgtgcccaggagg

SEQ ID NO: 28688 - DNA, 28 bp, synthetic construct
  source 1..28: mol_type = other DNA
ttccttccgtgcccaggaggcgtaaagg

SEQ ID NO: 28689 - DNA, 28 bp, synthetic construct
  source 1..28: mol_type = other DNA
tgcctttacgcctcctgggcacggaagg

SEQ ID NO: 28690 - DNA, 28 bp, synthetic construct
  source 1..28: mol_type = other DNA
aaaatgcctttacgcctcctgggcacgg

SEQ ID NO: 28691 - DNA, 28 bp, synthetic construct
  source 1..28: mol_type = other DNA
ctaaaaaaatgcctttacgcctcctggg

SEQ ID NO: 28692 - DNA, 28 bp, synthetic construct
  source 1..28: mol_type = other DNA
actaaaaaaatgcctttacgcctcctgg

SEQ ID NO: 28693 - DNA, 28 bp, synthetic construct
  source 1..28: mol_type = other DNA
gtcattctcattatctcttctatcttgg

SEQ ID NO: 28694 - DNA, 28 bp, synthetic construct
  source 1..28: mol_type = other DNA
tcattctcattatctcttctatcttggg

SEQ ID NO: 28695 - DNA, 28 bp, synthetic construct
  source 1..28: mol_type = other DNA
tggaaagggtagaataaacatggttagg

SEQ ID NO: 28696 - DNA, 28 bp, synthetic construct
  source 1..28: mol_type = other DNA
taagttggaaagggtagaataaacatgg

SEQ ID NO: 28697 - DNA, 28 bp, synthetic construct
  source 1..28: mol_type = other DNA
ggaaaaatgatctttaagttggaaaggg

SEQ ID NO: 28698 - DNA, 28 bp, synthetic construct
  source 1..28: mol_type = other DNA
aggaaaaatgatctttaagttggaaagg

SEQ ID NO: 28699 - DNA, 28 bp, synthetic construct
  source 1..28: mol_type = other DNA
ttatcaggaaaaatgatctttaagttgg

SEQ ID NO: 28700 - DNA, 28 bp, synthetic construct
  source 1..28: mol_type = other DNA
ctattttgattttatcatctttatcagg

SEQ ID NO: 28701 - DNA, 28 bp, synthetic construct
  source 1..28: mol_type = other DNA
gatggtatagagtaaacaaatgacatgg

SEQ ID NO: 28702 - DNA, 28 bp, synthetic construct
  source 1..28: mol_type = other DNA
tactctataccatctgttctaaataagg

SEQ ID NO: 28703 - DNA, 28 bp, synthetic construct
  source 1..28: mol_type = other DNA
aggacatagccttatttagaacagatgg

SEQ ID NO: 28704 - DNA, 28 bp, synthetic construct
  source 1..28: mol_type = other DNA
ctaaataaggctatgtccttttttgtgg

SEQ ID NO: 28705 - DNA, 28 bp, synthetic construct
  source 1..28: mol_type = other DNA
taaataaggctatgtccttttttgtggg

SEQ ID NO: 28706 - DNA, 28 bp, synthetic construct
  source 1..28: mol_type = other DNA
aaataaggctatgtccttttttgtgggg

SEQ ID NO: 28707 - DNA, 28 bp, synthetic construct
  source 1..28: mol_type = other DNA
ctatttggagcactccccacaaaaaagg

SEQ ID NO: 28708 - DNA, 28 bp, synthetic construct
  source 1..28: mol_type = other DNA
ataagagttttaaaacaatactatttgg

SEQ ID NO: 28709 - DNA, 28 bp, synthetic construct
  source 1..28: mol_type = other DNA
gtattgttttaaaactcttatatacagg

SEQ ID NO: 28710 - DNA, 28 bp, synthetic construct
  source 1..28: mol_type = other DNA
cttatatacaggcaaccacactttctgg

SEQ ID NO: 28711 - DNA, 28 bp, synthetic construct
  source 1..28: mol_type = other DNA
gcaaccacactttctggttcacctcagg

SEQ ID NO: 28712 - DNA, 28 bp, synthetic construct
  source 1..28: mol_type = other DNA
agtgcctgaggtgaaccagaaagtgtgg

SEQ ID NO: 28713 - DNA, 28 bp, synthetic construct
  source 1..28: mol_type = other DNA
actttctggttcacctcaggcactctgg

SEQ ID NO: 28714 - DNA, 28 bp, synthetic construct
  source 1..28: mol_type = other DNA
cagacagtatataccagagtgcctgagg

SEQ ID NO: 28715 - DNA, 28 bp, synthetic construct
  source 1..28: mol_type = other DNA
gcactctggtatatactgtctgccctgg

SEQ ID NO: 28716 - DNA, 28 bp, synthetic construct
  source 1..28: mol_type = other DNA
cactctggtatatactgtctgccctggg

SEQ ID NO: 28717 - DNA, 28 bp, synthetic construct
  source 1..28: mol_type = other DNA
actctggtatatactgtctgccctgggg

SEQ ID NO: 28718 - DNA, 28 bp, synthetic construct
  source 1..28: mol_type = other DNA
tctgccctggggtaaatacgaatagagg

SEQ ID NO: 28719 - DNA, 28 bp, synthetic construct
  source 1..28: mol_type = other DNA
gaggcctctattcgtatttaccccaggg

SEQ ID NO: 28720 - DNA, 28 bp, synthetic construct
  source 1..28: mol_type = other DNA
agaggcctctattcgtatttaccccagg

SEQ ID NO: 28721 - DNA, 28 bp, synthetic construct
  source 1..28: mol_type = other DNA
aggcctctttactctgaaaagtgtctgg

SEQ ID NO: 28722 - DNA, 28 bp, synthetic construct
  source 1..28: mol_type = other DNA
aaaccagacacttttcagagtaaagagg

SEQ ID NO: 28723 - DNA, 28 bp, synthetic construct
  source 1..28: mol_type = other DNA
aaaagtgtctggttttttgaacagctgg

SEQ ID NO: 28724 - DNA, 28 bp, synthetic construct
  source 1..28: mol_type = other DNA
ggttcaataagtaaagctgaagaaatgg

SEQ ID NO: 28725 - DNA, 28 bp, synthetic construct
  source 1..28: mol_type = other DNA
ctgaagaaatggtaaagcactccacagg

SEQ ID NO: 28726 - DNA, 28 bp, synthetic construct
  source 1..28: mol_type = other DNA
tgaagaaatggtaaagcactccacaggg

SEQ ID NO: 28727 - DNA, 28 bp, synthetic construct
  source 1..28: mol_type = other DNA
atggtaaagcactccacagggttcatgg

SEQ ID NO: 28728 - DNA, 28 bp, synthetic construct
  source 1..28: mol_type = other DNA
tggtaaagcactccacagggttcatggg

SEQ ID NO: 28729 - DNA, 28 bp, synthetic construct
  source 1..28: mol_type = other DNA
cactccacagggttcatgggctctcagg

SEQ ID NO: 28730 - DNA, 28 bp, synthetic construct
  source 1..28: mol_type = other DNA
aagacctgagagcccatgaaccctgtgg

SEQ ID NO: 28731 - DNA, 28 bp, synthetic construct
  source 1..28: mol_type = other DNA
tagttttctctttttcttgaatgtgtgg

SEQ ID NO: 28732 - DNA, 28 bp, synthetic construct
  source 1..28: mol_type = other DNA
agaaaactatttctgttgaaaactttgg

SEQ ID NO: 28733 - DNA, 28 bp, synthetic construct
  source 1..28: mol_type = other DNA
tttctgttgaaaactttggccacactgg

SEQ ID NO: 28734 - DNA, 28 bp, synthetic construct
  source 1..28: mol_type = other DNA
ttctgttgaaaactttggccacactggg

SEQ ID NO: 28735 - DNA, 28 bp, synthetic construct
  source 1..28: mol_type = other DNA
ttgaaaactttggccacactgggccagg

SEQ ID NO: 28736 - DNA, 28 bp, synthetic construct
  source 1..28: mol_type = other DNA
aactttggccacactgggccaggcatgg

SEQ ID NO: 28737 - DNA, 28 bp, synthetic construct
  source 1..28: mol_type = other DNA
aggtgtgaccatgcctggcccagtgtgg

SEQ ID NO: 28738 - DNA, 28 bp, synthetic construct
  source 1..28: mol_type = other DNA
ctgggattacaggtgtgaccatgcctgg

SEQ ID NO: 28739 - DNA, 28 bp, synthetic construct
  source 1..28: mol_type = other DNA
ggtcacacctgtaatcccagaactttgg

SEQ ID NO: 28740 - DNA, 28 bp, synthetic construct
  source 1..28: mol_type = other DNA
gtcacacctgtaatcccagaactttggg

SEQ ID NO: 28741 - DNA, 28 bp, synthetic construct
  source 1..28: mol_type = other DNA
tggcttcccaaagttctgggattacagg

SEQ ID NO: 28742 - DNA, 28 bp, synthetic construct
  source 1..28: mol_type = other DNA
atcccagaactttgggaagccaagacgg

SEQ ID NO: 28743 - DNA, 28 bp, synthetic construct
  source 1..28: mol_type = other DNA
tcccagaactttgggaagccaagacggg

SEQ ID NO: 28744 - DNA, 28 bp, synthetic construct
  source 1..28: mol_type = other DNA
acccgtcttggcttcccaaagttctggg

SEQ ID NO: 28745 - DNA, 28 bp, synthetic construct
  source 1..28: mol_type = other DNA
cacccgtcttggcttcccaaagttctgg

SEQ ID NO: 28746 - DNA, 28 bp, synthetic construct
  source 1..28: mol_type = other DNA
cagaactttgggaagccaagacgggtgg

SEQ ID NO: 28747 - DNA, 28 bp, synthetic construct
  source 1..28: mol_type = other DNA
ctgatctcaggtgatccacccgtcttgg

SEQ ID NO: 28748 - DNA, 28 bp, synthetic construct
  source 1..28: mol_type = other DNA
caagacgggtggatcacctgagatcagg

SEQ ID NO: 28749 - DNA, 28 bp, synthetic construct
  source 1..28: mol_type = other DNA
acgctggtctcgaactcctgatctcagg

SEQ ID NO: 28750 - DNA, 28 bp, synthetic construct
  source 1..28: mol_type = other DNA
tgagatcaggagttcgagaccagcgtgg

SEQ ID NO: 28751 - DNA, 28 bp, synthetic construct
  source 1..28: mol_type = other DNA
gagttcgagaccagcgtggccaacacgg

SEQ ID NO: 28752 - DNA, 28 bp, synthetic construct
  source 1..28: mol_type = other DNA
cagagtttcaccgtgttggccacgctgg

SEQ ID NO: 28753 - DNA, 28 bp, synthetic construct
  source 1..28: mol_type = other DNA
tggttgagacagagtttcaccgtgttgg

SEQ ID NO: 28754 - DNA, 28 bp, synthetic construct
  source 1..28: mol_type = other DNA
tcaaccaaaaatacaaaaattagccagg

SEQ ID NO: 28755 - DNA, 28 bp, synthetic construct
  source 1..28: mol_type = other DNA
catgcctggctaatttttgtatttttgg

SEQ ID NO: 28756 - DNA, 28 bp, synthetic construct
  source 1..28: mol_type = other DNA
caaaaatacaaaaattagccaggcatgg

SEQ ID NO: 28757 - DNA, 28 bp, synthetic construct
  source 1..28: mol_type = other DNA
aaatacaaaaattagccaggcatggtgg

SEQ ID NO: 28758 - DNA, 28 bp, synthetic construct
  source 1..28: mol_type = other DNA
tacaaaaattagccaggcatggtggcgg

SEQ ID NO: 28759 - DNA, 28 bp, synthetic construct
  source 1..28: mol_type = other DNA
acaaaaattagccaggcatggtggcggg

SEQ ID NO: 28760 - DNA, 28 bp, synthetic construct
  source 1..28: mol_type = other DNA
gattacaggcgcccgccaccatgcctgg

SEQ ID NO: 28761 - DNA, 28 bp, synthetic construct
  source 1..28: mol_type = other DNA
cgggcgcctgtaatcccagctactcagg

SEQ ID NO: 28762 - DNA, 28 bp, synthetic construct
  source 1..28: mol_type = other DNA
gcgcctgtaatcccagctactcaggagg

SEQ ID NO: 28763 - DNA, 28 bp, synthetic construct
  source 1..28: mol_type = other DNA
cagcctcctgagtagctgggattacagg

SEQ ID NO: 28764 - DNA, 28 bp, synthetic construct
  source 1..28: mol_type = other DNA
gtaatcccagctactcaggaggctgagg

SEQ ID NO: 28765 - DNA, 28 bp, synthetic construct
  source 1..28: mol_type = other DNA
tcccagctactcaggaggctgaggcagg

SEQ ID NO: 28766 - DNA, 28 bp, synthetic construct
  source 1..28: mol_type = other DNA
tcctgcctcagcctcctgagtagctggg

SEQ ID NO: 28767 - DNA, 28 bp, synthetic construct
  source 1..28: mol_type = other DNA
ctcctgcctcagcctcctgagtagctgg

SEQ ID NO: 28768 - DNA, 28 bp, synthetic construct
  source 1..28: mol_type = other DNA
caggaggctgaggcaggagaatcactgg

SEQ ID NO: 28769 - DNA, 28 bp, synthetic construct
  source 1..28: mol_type = other DNA
ctgaggcaggagaatcactggaactcgg

SEQ ID NO: 28770 - DNA, 28 bp, synthetic construct
  source 1..28: mol_type = other DNA
tgaggcaggagaatcactggaactcggg

SEQ ID NO: 28771 - DNA, 28 bp, synthetic construct
  source 1..28: mol_type = other DNA
ggcaggagaatcactggaactcgggagg

SEQ ID NO: 28772 - DNA, 28 bp, synthetic construct
  source 1..28: mol_type = other DNA
agaatcactggaactcgggaggcagagg

SEQ ID NO: 28773 - DNA, 28 bp, synthetic construct
  source 1..28: mol_type = other DNA
gagatcacgccactgcacaccagcctgg

SEQ ID NO: 28774 - DNA, 28 bp, synthetic construct
  source 1..28: mol_type = other DNA
agatcacgccactgcacaccagcctggg

SEQ ID NO: 28775 - DNA, 28 bp, synthetic construct
  source 1..28: mol_type = other DNA
ctctgttgcccaggctggtgtgcagtgg

SEQ ID NO: 28776 - DNA, 28 bp, synthetic construct
  source 1..28: mol_type = other DNA
cagagtcttgctctgttgcccaggctgg

SEQ ID NO: 28777 - DNA, 28 bp, synthetic construct
  source 1..28: mol_type = other DNA
gagacagagtcttgctctgttgcccagg

SEQ ID NO: 28778 - DNA, 28 bp, synthetic construct
  source 1..28: mol_type = other DNA
aaaaaaaaaaaaactctagccacactgg

SEQ ID NO: 28779 - DNA, 28 bp, synthetic construct
  source 1..28: mol_type = other DNA
tctagccacactggattcatatcctagg

SEQ ID NO: 28780 - DNA, 28 bp, synthetic construct
  source 1..28: mol_type = other DNA
gcaggcctaggatatgaatccagtgtgg

SEQ ID NO: 28781 - DNA, 28 bp, synthetic construct
  source 1..28: mol_type = other DNA
catagaactagtaagtggcaggcctagg

SEQ ID NO: 28782 - DNA, 28 bp, synthetic construct
  source 1..28: mol_type = other DNA
tgtggtcatagaactagtaagtggcagg

SEQ ID NO: 28783 - DNA, 28 bp, synthetic construct
  source 1..28: mol_type = other DNA
tgccacttactagttctatgaccacagg

SEQ ID NO: 28784 - DNA, 28 bp, synthetic construct
  source 1..28: mol_type = other DNA
atcctgtggtcatagaactagtaagtgg

SEQ ID NO: 28785 - DNA, 28 bp, synthetic construct
  source 1..28: mol_type = other DNA
taaagagattgggtaacttatcctgtgg

SEQ ID NO: 28786 - DNA, 28 bp, synthetic construct
  source 1..28: mol_type = other DNA
agttgagctgagagttaaagagattggg

SEQ ID NO: 28787 - DNA, 28 bp, synthetic construct
  source 1..28: mol_type = other DNA
gagttgagctgagagttaaagagattgg

SEQ ID NO: 28788 - DNA, 28 bp, synthetic construct
  source 1..28: mol_type = other DNA
ctctttaactctcagctcaactcactgg

SEQ ID NO: 28789 - DNA, 28 bp, synthetic construct
  source 1..28: mol_type = other DNA
tttaatcatgcatttagtattaaatagg

SEQ ID NO: 28790 - DNA, 28 bp, synthetic construct
  source 1..28: mol_type = other DNA
tgatagtaatattggcaatgataattgg

SEQ ID NO: 28791 - DNA, 28 bp, synthetic construct
  source 1..28: mol_type = other DNA
gagttaataacactgatagtaatattgg

SEQ ID NO: 28792 - DNA, 28 bp, synthetic construct
  source 1..28: mol_type = other DNA
ctccctcaacccctccacagcaacatgg

SEQ ID NO: 28793 - DNA, 28 bp, synthetic construct
  source 1..28: mol_type = other DNA
taccatgttgctgtggaggggttgaggg

SEQ ID NO: 28794 - DNA, 28 bp, synthetic construct
  source 1..28: mol_type = other DNA
ataccatgttgctgtggaggggttgagg

SEQ ID NO: 28795 - DNA, 28 bp, synthetic construct
  source 1..28: mol_type = other DNA
tcacagataccatgttgctgtggagggg

SEQ ID NO: 28796 - DNA, 28 bp, synthetic construct
  source 1..28: mol_type = other DNA
gtcacagataccatgttgctgtggaggg

SEQ ID NO: 28797 - DNA, 28 bp, synthetic construct
  source 1..28: mol_type = other DNA
agtcacagataccatgttgctgtggagg

SEQ ID NO: 28798 - DNA, 28 bp, synthetic construct
  source 1..28: mol_type = other DNA
gagagtcacagataccatgttgctgtgg

SEQ ID NO: 28799 - DNA, 28 bp, synthetic construct
  source 1..28: mol_type = other DNA
caacatggtatctgtgactctctattgg

SEQ ID NO: 28800 - DNA, 28 bp, synthetic construct
  source 1..28: mol_type = other DNA
acaagatgtgacattctgaaaaggaagg

SEQ ID NO: 28801 - DNA, 28 bp, synthetic construct
  source 1..28: mol_type = other DNA
gaaaacaagatgtgacattctgaaaagg

SEQ ID NO: 28802 - DNA, 28 bp, synthetic construct
  source 1..28: mol_type = other DNA
tgttttctcaccaatctcttgctactgg

SEQ ID NO: 28803 - DNA, 28 bp, synthetic construct
  source 1..28: mol_type = other DNA
tgagtttaaaccagtagcaagagattgg

SEQ ID NO: 28804 - DNA, 28 bp, synthetic construct
  source 1..28: mol_type = other DNA
agaaagactttacgagattgtggggagg

SEQ ID NO: 28805 - DNA, 28 bp, synthetic construct
  source 1..28: mol_type = other DNA
atgagaaagactttacgagattgtgggg

SEQ ID NO: 28806 - DNA, 28 bp, synthetic construct
  source 1..28: mol_type = other DNA
gatgagaaagactttacgagattgtggg

SEQ ID NO: 28807 - DNA, 28 bp, synthetic construct
  source 1..28: mol_type = other DNA
agatgagaaagactttacgagattgtgg

SEQ ID NO: 28808 - DNA, 28 bp, synthetic construct
  source 1..28: mol_type = other DNA
gaaatctttgtcttcactagaaatctgg

SEQ ID NO: 28809 - DNA, 28 bp, synthetic construct
  source 1..28: mol_type = other DNA
ttcactagaaatctggaatactccaagg

SEQ ID NO: 28810 - DNA, 28 bp, synthetic construct
  source 1..28: mol_type = other DNA
gaatactccaaggaagtttcttctctgg

SEQ ID NO: 28811 - DNA, 28 bp, synthetic construct
  source 1..28: mol_type = other DNA
ttctttgccagagaagaaacttccttgg

SEQ ID NO: 28812 - DNA, 28 bp, synthetic construct
  source 1..28: mol_type = other DNA
cacaaattatgtttgttataaatgctgg

SEQ ID NO: 28813 - DNA, 28 bp, synthetic construct
  source 1..28: mol_type = other DNA
aacaaacataatttgtgagctgctctgg

SEQ ID NO: 28814 - DNA, 28 bp, synthetic construct
  source 1..28: mol_type = other DNA
ggaaagacagttgctgagggattcatgg

SEQ ID NO: 28815 - DNA, 28 bp, synthetic construct
  source 1..28: mol_type = other DNA
tgaatccctcagcaactgtctttcctgg

SEQ ID NO: 28816 - DNA, 28 bp, synthetic construct
  source 1..28: mol_type = other DNA
tgattccaggaaagacagttgctgaggg

SEQ ID NO: 28817 - DNA, 28 bp, synthetic construct
  source 1..28: mol_type = other DNA
ttgattccaggaaagacagttgctgagg

SEQ ID NO: 28818 - DNA, 28 bp, synthetic construct
  source 1..28: mol_type = other DNA
aagaataatagtttatcttgattccagg

SEQ ID NO: 28819 - DNA, 28 bp, synthetic construct
  source 1..28: mol_type = other DNA
aatcaagataaactattattcttcatgg

SEQ ID NO: 28820 - DNA, 28 bp, synthetic construct
  source 1..28: mol_type = other DNA
aaactattattcttcatggttcccttgg

SEQ ID NO: 28821 - DNA, 28 bp, synthetic construct
  source 1..28: mol_type = other DNA
aactattattcttcatggttcccttggg

SEQ ID NO: 28822 - DNA, 28 bp, synthetic construct
  source 1..28: mol_type = other DNA
ctaagttttcagagtgtgttcccaaggg

SEQ ID NO: 28823 - DNA, 28 bp, synthetic construct
  source 1..28: mol_type = other DNA
ccttgggaacacactctgaaaacttagg

SEQ ID NO: 28824 - DNA, 28 bp, synthetic construct
  source 1..28: mol_type = other DNA
ttaatgtcattttattttctagctaggg

SEQ ID NO: 28825 - DNA, 28 bp, synthetic construct
  source 1..28: mol_type = other DNA
gttaatgtcattttattttctagctagg

SEQ ID NO: 28826 - DNA, 28 bp, synthetic construct
  source 1..28: mol_type = other DNA
aaaatgacattaactttctgagaaaagg

SEQ ID NO: 28827 - DNA, 28 bp, synthetic construct
  source 1..28: mol_type = other DNA
actttctgagaaaaggactgacccaagg

SEQ ID NO: 28828 - DNA, 28 bp, synthetic construct
  source 1..28: mol_type = other DNA
ggactgacccaaggcatattcaaatagg

SEQ ID NO: 28829 - DNA, 28 bp, synthetic construct
  source 1..28: mol_type = other DNA
gactgacccaaggcatattcaaataggg

SEQ ID NO: 28830 - DNA, 28 bp, synthetic construct
  source 1..28: mol_type = other DNA
actgacccaaggcatattcaaatagggg

SEQ ID NO: 28831 - DNA, 28 bp, synthetic construct
  source 1..28: mol_type = other DNA
tgattcccctatttgaatatgccttggg

SEQ ID NO: 28832 - DNA, 28 bp, synthetic construct
  source 1..28: mol_type = other DNA
atgattcccctatttgaatatgccttgg

SEQ ID NO: 28833 - DNA, 28 bp, synthetic construct
  source 1..28: mol_type = other DNA
catattcaaataggggaatcataaaagg

SEQ ID NO: 28834 - DNA, 28 bp, synthetic construct
  source 1..28: mol_type = other DNA
atattcaaataggggaatcataaaaggg

SEQ ID NO: 28835 - DNA, 28 bp, synthetic construct
  source 1..28: mol_type = other DNA
aggggaatcataaaagggaccacacagg

SEQ ID NO: 28836 - DNA, 28 bp, synthetic construct
  source 1..28: mol_type = other DNA
agctatcactcatttttctcctgtgtgg

SEQ ID NO: 28837 - DNA, 28 bp, synthetic construct
  source 1..28: mol_type = other DNA
tggcatatcttagttactcagtaaatgg

SEQ ID NO: 28838 - DNA, 28 bp, synthetic construct
  source 1..28: mol_type = other DNA
tgagtaactaagatatgccaagaaatgg

SEQ ID NO: 28839 - DNA, 28 bp, synthetic construct
  source 1..28: mol_type = other DNA
aagatatgccaagaaatggcataccagg

SEQ ID NO: 28840 - DNA, 28 bp, synthetic construct
  source 1..28: mol_type = other DNA
ataaaatgcctggtatgccatttcttgg

SEQ ID NO: 28841 - DNA, 28 bp, synthetic construct
  source 1..28: mol_type = other DNA
catgaaatcatgtttataaaatgcctgg

SEQ ID NO: 28842 - DNA, 28 bp, synthetic construct
  source 1..28: mol_type = other DNA
caggcattttataaacatgatttcatgg

SEQ ID NO: 28843 - DNA, 28 bp, synthetic construct
  source 1..28: mol_type = other DNA
catggattcttctcaacaattttgctgg

SEQ ID NO: 28844 - DNA, 28 bp, synthetic construct
  source 1..28: mol_type = other DNA
ttctcaacaattttgctggaaattgagg

SEQ ID NO: 28845 - DNA, 28 bp, synthetic construct
  source 1..28: mol_type = other DNA
aattttgctggaaattgaggctcagagg

SEQ ID NO: 28846 - DNA, 28 bp, synthetic construct
  source 1..28: mol_type = other DNA
gaggctcagaggaagcacttgcccaagg

SEQ ID NO: 28847 - DNA, 28 bp, synthetic construct
  source 1..28: mol_type = other DNA
aggctcagaggaagcacttgcccaaggg

SEQ ID NO: 28848 - DNA, 28 bp, synthetic construct
  source 1..28: mol_type = other DNA
ttgcccaagggacataactagtaaatgg

SEQ ID NO: 28849 - DNA, 28 bp, synthetic construct
  source 1..28: mol_type = other DNA
ctgccatttactagttatgtcccttggg

SEQ ID NO: 28850 - DNA, 28 bp, synthetic construct
  source 1..28: mol_type = other DNA
ccaagggacataactagtaaatggcagg

SEQ ID NO: 28851 - DNA, 28 bp, synthetic construct
  source 1..28: mol_type = other DNA
taaatggcaggtacagcacttaccacgg

SEQ ID NO: 28852 - DNA, 28 bp, synthetic construct
  source 1..28: mol_type = other DNA
aaatggcaggtacagcacttaccacggg

SEQ ID NO: 28853 - DNA, 28 bp, synthetic construct
  source 1..28: mol_type = other DNA
ttgaacttagagtgcagaagacccgtgg

SEQ ID NO: 28854 - DNA, 28 bp, synthetic construct
  source 1..28: mol_type = other DNA
cttcagtaaaaaaatacacgtagcatgg

SEQ ID NO: 28855 - DNA, 28 bp, synthetic construct
  source 1..28: mol_type = other DNA
catgctacgtgtatttttttactgaagg

SEQ ID NO: 28856 - DNA, 28 bp, synthetic construct
  source 1..28: mol_type = other DNA
tttttaactgtctcaaaaactagtttgg

SEQ ID NO: 28857 - DNA, 28 bp, synthetic construct
  source 1..28: mol_type = other DNA
agtttttgagacagttaaaaataaaagg

SEQ ID NO: 28858 - DNA, 28 bp, synthetic construct
  source 1..28: mol_type = other DNA
agaaaaaaaaatatataaacattgttgg

SEQ ID NO: 28859 - DNA, 28 bp, synthetic construct
  source 1..28: mol_type = other DNA
aaatatataaacattgttggttaagtgg

SEQ ID NO: 28860 - DNA, 28 bp, synthetic construct
  source 1..28: mol_type = other DNA
ttcatcattcaaaattgctaattaaagg

SEQ ID NO: 28861 - DNA, 28 bp, synthetic construct
  source 1..28: mol_type = other DNA
attttgaatgatgaaacagccacatagg

SEQ ID NO: 28862 - DNA, 28 bp, synthetic construct
  source 1..28: mol_type = other DNA
aacagccacataggtgcaatgcttctgg

SEQ ID NO: 28863 - DNA, 28 bp, synthetic construct
  source 1..28: mol_type = other DNA
cctggccagaagcattgcacctatgtgg

SEQ ID NO: 28864 - DNA, 28 bp, synthetic construct
  source 1..28: mol_type = other DNA
cacataggtgcaatgcttctggccaggg

SEQ ID NO: 28865 - DNA, 28 bp, synthetic construct
  source 1..28: mol_type = other DNA
atgcttctggccagggcagctcattagg

SEQ ID NO: 28866 - DNA, 28 bp, synthetic construct
  source 1..28: mol_type = other DNA
tgcttctggccagggcagctcattaggg

SEQ ID NO: 28867 - DNA, 28 bp, synthetic construct
  source 1..28: mol_type = other DNA
atactgagtccctaatgagctgccctgg

SEQ ID NO: 28868 - DNA, 28 bp, synthetic construct
  source 1..28: mol_type = other DNA
agtatccgaagtctttctttttttttgg

SEQ ID NO: 28869 - DNA, 28 bp, synthetic construct
  source 1..28: mol_type = other DNA
tccgaagtctttctttttttttggatgg

SEQ ID NO: 28870 - DNA, 28 bp, synthetic construct
  source 1..28: mol_type = other DNA
gccatccaaaaaaaaagaaagacttcgg

SEQ ID NO: 28871 - DNA, 28 bp, synthetic construct
  source 1..28: mol_type = other DNA
gtagaggctatacagtgtgtatacatgg

SEQ ID NO: 28872 - DNA, 28 bp, synthetic construct
  source 1..28: mol_type = other DNA
gctaagtggtatgtaattttggtagagg

SEQ ID NO: 28873 - DNA, 28 bp, synthetic construct
  source 1..28: mol_type = other DNA
attcgtgctaagtggtatgtaattttgg

SEQ ID NO: 28874 - DNA, 28 bp, synthetic construct
  source 1..28: mol_type = other DNA
agggatctcttgcattcgtgctaagtgg

SEQ ID NO: 28875 - DNA, 28 bp, synthetic construct
  source 1..28: mol_type = other DNA
taatttttgtttatagtacgaggaaggg

SEQ ID NO: 28876 - DNA, 28 bp, synthetic construct
  source 1..28: mol_type = other DNA
ttaatttttgtttatagtacgaggaagg

SEQ ID NO: 28877 - DNA, 28 bp, synthetic construct
  source 1..28: mol_type = other DNA
tgagttaatttttgtttatagtacgagg

SEQ ID NO: 28878 - DNA, 28 bp, synthetic construct
  source 1..28: mol_type = other DNA
ttttatagttttgtctcttacatttagg

SEQ ID NO: 28879 - DNA, 28 bp, synthetic construct
  source 1..28: mol_type = other DNA
aaactataaaactcttagaaaatatagg

SEQ ID NO: 28880 - DNA, 28 bp, synthetic construct
  source 1..28: mol_type = other DNA
atatctaagaaggttttgctaatcaagg

SEQ ID NO: 28881 - DNA, 28 bp, synthetic construct
  source 1..28: mol_type = other DNA
tgtacttttcgtgtcatatctaagaagg

SEQ ID NO: 28882 - DNA, 28 bp, synthetic construct
  source 1..28: mol_type = other DNA
gtgtatcttttcaatttcttgataatgg

SEQ ID NO: 28883 - DNA, 28 bp, synthetic construct
  source 1..28: mol_type = other DNA
agaaattgaaaagatacacacagaatgg

SEQ ID NO: 28884 - DNA, 28 bp, synthetic construct
  source 1..28: mol_type = other DNA
gaaattgaaaagatacacacagaatggg

SEQ ID NO: 28885 - DNA, 28 bp, synthetic construct
  source 1..28: mol_type = other DNA
atatctgtaaatcatgtatctgataagg

SEQ ID NO: 28886 - DNA, 28 bp, synthetic construct
  source 1..28: mol_type = other DNA
tatctgtaaatcatgtatctgataaggg

SEQ ID NO: 28887 - DNA, 28 bp, synthetic construct
  source 1..28: mol_type = other DNA
gttgtaagaattcagtgtatatttcagg

SEQ ID NO: 28888 - DNA, 28 bp, synthetic construct
  source 1..28: mol_type = other DNA
caagaatgtttgctcattttaaaatagg

SEQ ID NO: 28889 - DNA, 28 bp, synthetic construct
  source 1..28: mol_type = other DNA
ctattttaaaatgagcaaacattcttgg

SEQ ID NO: 28890 - DNA, 28 bp, synthetic construct
  source 1..28: mol_type = other DNA
ttaaaatgagcaaacattcttggccagg

SEQ ID NO: 28891 - DNA, 28 bp, synthetic construct
  source 1..28: mol_type = other DNA
agcaaacattcttggccaggtgcaatgg

SEQ ID NO: 28892 - DNA, 28 bp, synthetic construct
  source 1..28: mol_type = other DNA
gattacatgcatgagccattgcacctgg

SEQ ID NO: 28893 - DNA, 28 bp, synthetic construct
  source 1..28: mol_type = other DNA
gctcatgcatgtaatcccagcactttgg

SEQ ID NO: 28894 - DNA, 28 bp, synthetic construct
  source 1..28: mol_type = other DNA
ctcatgcatgtaatcccagcactttggg

SEQ ID NO: 28895 - DNA, 28 bp, synthetic construct
  source 1..28: mol_type = other DNA
atgcatgtaatcccagcactttgggagg

SEQ ID NO: 28896 - DNA, 28 bp, synthetic construct
  source 1..28: mol_type = other DNA
gtaatcccagcactttgggaggccaagg

SEQ ID NO: 28897 - DNA, 28 bp, synthetic construct
  source 1..28: mol_type = other DNA
taatcccagcactttgggaggccaaggg

SEQ ID NO: 28898 - DNA, 28 bp, synthetic construct
  source 1..28: mol_type = other DNA
tcccagcactttgggaggccaagggagg

SEQ ID NO: 28899 - DNA, 28 bp, synthetic construct
  source 1..28: mol_type = other DNA
acctcccttggcctcccaaagtgctggg

SEQ ID NO: 28900 - DNA, 28 bp, synthetic construct
  source 1..28: mol_type = other DNA
cacctcccttggcctcccaaagtgctgg

SEQ ID NO: 28901 - DNA, 28 bp, synthetic construct
  source 1..28: mol_type = other DNA
cagcactttgggaggccaagggaggtgg

SEQ ID NO: 28902 - DNA, 28 bp, synthetic construct
  source 1..28: mol_type = other DNA
gaggccaagggaggtggatcacttgagg

SEQ ID NO: 28903 - DNA, 28 bp, synthetic construct
  source 1..28: mol_type = other DNA
ctgacctcaagtgatccacctcccttgg

SEQ ID NO: 28904 - DNA, 28 bp, synthetic construct
  source 1..28: mol_type = other DNA
caagggaggtggatcacttgaggtcagg

SEQ ID NO: 28905 - DNA, 28 bp, synthetic construct
  source 1..28: mol_type = other DNA
tgaggtcaggagttcaagaccagcctgg

SEQ ID NO: 28906 - DNA, 28 bp, synthetic construct
  source 1..28: mol_type = other DNA
gagttcaagaccagcctggccaacatgg

SEQ ID NO: 28907 - DNA, 28 bp, synthetic construct
  source 1..28: mol_type = other DNA
tggggtttcaccatgttggccaggctgg

SEQ ID NO: 28908 - DNA, 28 bp, synthetic construct
  source 1..28: mol_type = other DNA
gagatggggtttcaccatgttggccagg

SEQ ID NO: 28909 - DNA, 28 bp, synthetic construct
  source 1..28: mol_type = other DNA
taatagagatggggtttcaccatgttgg

SEQ ID NO: 28910 - DNA, 28 bp, synthetic construct
  source 1..28: mol_type = other DNA
aatttttgtatttttaatagagatgggg

SEQ ID NO: 28911 - DNA, 28 bp, synthetic construct
  source 1..28: mol_type = other DNA
taatttttgtatttttaatagagatggg

SEQ ID NO: 28912 - DNA, 28 bp, synthetic construct
  source 1..28: mol_type = other DNA
ctaatttttgtatttttaatagagatgg

SEQ ID NO: 28913 - DNA, 28 bp, synthetic construct
  source 1..28: mol_type = other DNA
tctattaaaaatacaaaaattagccagg

SEQ ID NO: 28914 - DNA, 28 bp, synthetic construct
  source 1..28: mol_type = other DNA
taaaaatacaaaaattagccaggcttgg

SEQ ID NO: 28915 - DNA, 28 bp, synthetic construct
  source 1..28: mol_type = other DNA
aaatacaaaaattagccaggcttggtgg

SEQ ID NO: 28916 - DNA, 28 bp, synthetic construct
  source 1..28: mol_type = other DNA
tacaaaaattagccaggcttggtggtgg

SEQ ID NO: 28917 - DNA, 28 bp, synthetic construct
  source 1..28: mol_type = other DNA
acaaaaattagccaggcttggtggtggg

SEQ ID NO: 28918 - DNA, 28 bp, synthetic construct
  source 1..28: mol_type = other DNA
gattacaggcacccaccaccaagcctgg

SEQ ID NO: 28919 - DNA, 28 bp, synthetic construct
  source 1..28: mol_type = other DNA
gtgggtgcctgtaatctcagctacttgg

SEQ ID NO: 28920 - DNA, 28 bp, synthetic construct
  source 1..28: mol_type = other DNA
tgggtgcctgtaatctcagctacttggg

SEQ ID NO: 28921 - DNA, 28 bp, synthetic construct
  source 1..28: mol_type = other DNA
gtgcctgtaatctcagctacttgggagg

SEQ ID NO: 28922 - DNA, 28 bp, synthetic construct
  source 1..28: mol_type = other DNA
cagcctcccaagtagctgagattacagg

SEQ ID NO: 28923 - DNA, 28 bp, synthetic construct
  source 1..28: mol_type = other DNA
gtaatctcagctacttgggaggctgagg

SEQ ID NO: 28924 - DNA, 28 bp, synthetic construct
  source 1..28: mol_type = other DNA
tctcagctacttgggaggctgaggcagg

SEQ ID NO: 28925 - DNA, 28 bp, synthetic construct
  source 1..28: mol_type = other DNA
ctgaggcaggagaatagcttgaacctgg

SEQ ID NO: 28926 - DNA, 28 bp, synthetic construct
  source 1..28: mol_type = other DNA
tgaggcaggagaatagcttgaacctggg

SEQ ID NO: 28927 - DNA, 28 bp, synthetic construct
  source 1..28: mol_type = other DNA
ggcaggagaatagcttgaacctgggagg

SEQ ID NO: 28928 - DNA, 28 bp, synthetic construct
  source 1..28: mol_type = other DNA
tggttcactgtaggctctgcctcccagg

SEQ ID NO: 28929 - DNA, 28 bp, synthetic construct
  source 1..28: mol_type = other DNA
cagtggcacgatcttggttcactgtagg

SEQ ID NO: 28930 - DNA, 28 bp, synthetic construct
  source 1..28: mol_type = other DNA
aggctggagtgcagtggcacgatcttgg

SEQ ID NO: 28931 - DNA, 28 bp, synthetic construct
  source 1..28: mol_type = other DNA
aagatcgtgccactgcactccagcctgg

SEQ ID NO: 28932 - DNA, 28 bp, synthetic construct
  source 1..28: mol_type = other DNA
agatcgtgccactgcactccagcctggg

SEQ ID NO: 28933 - DNA, 28 bp, synthetic construct
  source 1..28: mol_type = other DNA
ttctgttgcccaggctggagtgcagtgg

SEQ ID NO: 28934 - DNA, 28 bp, synthetic construct
  source 1..28: mol_type = other DNA
agagtctcacttctgttgcccaggctgg

SEQ ID NO: 28935 - DNA, 28 bp, synthetic construct
  source 1..28: mol_type = other DNA
agacagagtctcacttctgttgcccagg

SEQ ID NO: 28936 - DNA, 28 bp, synthetic construct
  source 1..28: mol_type = other DNA
ctttttttttttttttttttttttttgg

SEQ ID NO: 28937 - DNA, 28 bp, synthetic construct
  source 1..28: mol_type = other DNA
aaaaaaaaaaaaaaaaaaaaagcaatgg

SEQ ID NO: 28938 - DNA, 28 bp, synthetic construct
  source 1..28: mol_type = other DNA
catttctctaaagaagataaatgaatgg

SEQ ID NO: 28939 - DNA, 28 bp, synthetic construct
  source 1..28: mol_type = other DNA
agataaatgaatggcaaataagcacagg

SEQ ID NO: 28940 - DNA, 28 bp, synthetic construct
  source 1..28: mol_type = other DNA
atgaatggcaaataagcacaggaaaagg

SEQ ID NO: 28941 - DNA, 28 bp, synthetic construct
  source 1..28: mol_type = other DNA
aggtgttcaacatctttagtctttaagg

SEQ ID NO: 28942 - DNA, 28 bp, synthetic construct
  source 1..28: mol_type = other DNA
ctacatgtgtggtggtgtctcattgtgg

SEQ ID NO: 28943 - DNA, 28 bp, synthetic construct
  source 1..28: mol_type = other DNA
tgagacaccaccacacatgtagcattgg

SEQ ID NO: 28944 - DNA, 28 bp, synthetic construct
  source 1..28: mol_type = other DNA
gagacaccaccacacatgtagcattggg

SEQ ID NO: 28945 - DNA, 28 bp, synthetic construct
  source 1..28: mol_type = other DNA
aggcatcccaatgctacatgtgtggtgg

SEQ ID NO: 28946 - DNA, 28 bp, synthetic construct
  source 1..28: mol_type = other DNA
tataggcatcccaatgctacatgtgtgg

SEQ ID NO: 28947 - DNA, 28 bp, synthetic construct
  source 1..28: mol_type = other DNA
ttttaattatgtgtctttttgatatagg

SEQ ID NO: 28948 - DNA, 28 bp, synthetic construct
  source 1..28: mol_type = other DNA
gacacataattaaaaagtcttagtgagg

SEQ ID NO: 28949 - DNA, 28 bp, synthetic construct
  source 1..28: mol_type = other DNA
taattaaaaagtcttagtgaggctgtgg

SEQ ID NO: 28950 - DNA, 28 bp, synthetic construct
  source 1..28: mol_type = other DNA
agtcttagtgaggctgtggagaaactgg

SEQ ID NO: 28951 - DNA, 28 bp, synthetic construct
  source 1..28: mol_type = other DNA
aactggaaccttcatacaccactagtgg

SEQ ID NO: 28952 - DNA, 28 bp, synthetic construct
  source 1..28: mol_type = other DNA
actggaaccttcatacaccactagtggg

SEQ ID NO: 28953 - DNA, 28 bp, synthetic construct
  source 1..28: mol_type = other DNA
gtaaactcccactagtggtgtatgaagg

SEQ ID NO: 28954 - DNA, 28 bp, synthetic construct
  source 1..28: mol_type = other DNA
tcatacaccactagtgggagtttactgg

SEQ ID NO: 28955 - DNA, 28 bp, synthetic construct
  source 1..28: mol_type = other DNA
acaccactagtgggagtttactggtagg

SEQ ID NO: 28956 - DNA, 28 bp, synthetic construct
  source 1..28: mol_type = other DNA
caccactagtgggagtttactggtaggg

SEQ ID NO: 28957 - DNA, 28 bp, synthetic construct
  source 1..28: mol_type = other DNA
gaccctaccagtaaactcccactagtgg

SEQ ID NO: 28958 - DNA, 28 bp, synthetic construct
  source 1..28: mol_type = other DNA
gggtcgtaaagatattctaaaattatgg

SEQ ID NO: 28959 - DNA, 28 bp, synthetic construct
  source 1..28: mol_type = other DNA
taaagatattctaaaattatggtgatgg

SEQ ID NO: 28960 - DNA, 28 bp, synthetic construct
  source 1..28: mol_type = other DNA
catctatataaagtgtacaattcaatgg

SEQ ID NO: 28961 - DNA, 28 bp, synthetic construct
  source 1..28: mol_type = other DNA
ttgaattgtacactttatatagatgagg

SEQ ID NO: 28962 - DNA, 28 bp, synthetic construct
  source 1..28: mol_type = other DNA
gtacactttatatagatgaggtgtatgg

SEQ ID NO: 28963 - DNA, 28 bp, synthetic construct
  source 1..28: mol_type = other DNA
gaattatatctgaatatagccagcgtgg

SEQ ID NO: 28964 - DNA, 28 bp, synthetic construct
  source 1..28: mol_type = other DNA
attttctttaaaacaacaaccacgctgg

SEQ ID NO: 28965 - DNA, 28 bp, synthetic construct
  source 1..28: mol_type = other DNA
agcgtggttgttgttttaaagaaaatgg

SEQ ID NO: 28966 - DNA, 28 bp, synthetic construct
  source 1..28: mol_type = other DNA
tatgtcctcatttcttccaaatccaagg

SEQ ID NO: 28967 - DNA, 28 bp, synthetic construct
  source 1..28: mol_type = other DNA
acttgccttggatttggaagaaatgagg

SEQ ID NO: 28968 - DNA, 28 bp, synthetic construct
  source 1..28: mol_type = other DNA
ttccaaatccaaggcaagttagcaaagg

SEQ ID NO: 28969 - DNA, 28 bp, synthetic construct
  source 1..28: mol_type = other DNA
tgcctttgctaacttgccttggatttgg

SEQ ID NO: 28970 - DNA, 28 bp, synthetic construct
  source 1..28: mol_type = other DNA
tcattatgcctttgctaacttgccttgg

SEQ ID NO: 28971 - DNA, 28 bp, synthetic construct
  source 1..28: mol_type = other DNA
ttagcaaaggcataatgagaaaaagagg

SEQ ID NO: 28972 - DNA, 28 bp, synthetic construct
  source 1..28: mol_type = other DNA
aaaaagaggtctaattttcattcagagg

SEQ ID NO: 28973 - DNA, 28 bp, synthetic construct
  source 1..28: mol_type = other DNA
tcagaggccacatcagtgctccatctgg

SEQ ID NO: 28974 - DNA, 28 bp, synthetic construct
  source 1..28: mol_type = other DNA
tctttgtccagatggagcactgatgtgg

SEQ ID NO: 28975 - DNA, 28 bp, synthetic construct
  source 1..28: mol_type = other DNA
cttcttggctgactctttgtccagatgg

SEQ ID NO: 28976 - DNA, 28 bp, synthetic construct
  source 1..28: mol_type = other DNA
agagtcagccaagaagccaactgccagg

SEQ ID NO: 28977 - DNA, 28 bp, synthetic construct
  source 1..28: mol_type = other DNA
cagccaagaagccaactgccaggagtgg

SEQ ID NO: 28978 - DNA, 28 bp, synthetic construct
  source 1..28: mol_type = other DNA
cttccactcctggcagttggcttcttgg

SEQ ID NO: 28979 - DNA, 28 bp, synthetic construct
  source 1..28: mol_type = other DNA
gtggtcatcttccactcctggcagttgg

SEQ ID NO: 28980 - DNA, 28 bp, synthetic construct
  source 1..28: mol_type = other DNA
cctggaagtggtcatcttccactcctgg

SEQ ID NO: 28981 - DNA, 28 bp, synthetic construct
  source 1..28: mol_type = other DNA
gtggaagatgaccacttccaggatctgg

SEQ ID NO: 28982 - DNA, 28 bp, synthetic construct
  source 1..28: mol_type = other DNA
aagtctctctgccagatcctggaagtgg

SEQ ID NO: 28983 - DNA, 28 bp, synthetic construct
  source 1..28: mol_type = other DNA
cttgcaaagtctctctgccagatcctgg

SEQ ID NO: 28984 - DNA, 28 bp, synthetic construct
  source 1..28: mol_type = other DNA
gagactttgcaagtgcctttgaaagagg

SEQ ID NO: 28985 - DNA, 28 bp, synthetic construct
  source 1..28: mol_type = other DNA
atacattttcattgtcctctttcaaagg

SEQ ID NO: 28986 - DNA, 28 bp, synthetic construct
  source 1..28: mol_type = other DNA
tgaaagaggacaatgaaaatgtatctgg

SEQ ID NO: 28987 - DNA, 28 bp, synthetic construct
  source 1..28: mol_type = other DNA
aaatgtatctggcatgaaacacagcagg

SEQ ID NO: 28988 - DNA, 28 bp, synthetic construct
  source 1..28: mol_type = other DNA
tgaaacacagcaggatccaaagaacagg

SEQ ID NO: 28989 - DNA, 28 bp, synthetic construct
  source 1..28: mol_type = other DNA
actggcaatatcaaagcctgttctttgg

SEQ ID NO: 28990 - DNA, 28 bp, synthetic construct
  source 1..28: mol_type = other DNA
tgatcttaaagacacgcatcatgactgg

SEQ ID NO: 28991 - DNA, 28 bp, synthetic construct
  source 1..28: mol_type = other DNA
ggatcagaaggatacacttagtcatagg

SEQ ID NO: 28992 - DNA, 28 bp, synthetic construct
  source 1..28: mol_type = other DNA
tctaactgcacacgagtggatcagaagg

SEQ ID NO: 28993 - DNA, 28 bp, synthetic construct
  source 1..28: mol_type = other DNA
tgggtgttctctaactgcacacgagtgg

SEQ ID NO: 28994 - DNA, 28 bp, synthetic construct
  source 1..28: mol_type = other DNA
ctcgtgtgcagttagagaacacccaagg

SEQ ID NO: 28995 - DNA, 28 bp, synthetic construct
  source 1..28: mol_type = other DNA
tcgtgtgcagttagagaacacccaaggg

SEQ ID NO: 28996 - DNA, 28 bp, synthetic construct
  source 1..28: mol_type = other DNA
cgtgtgcagttagagaacacccaagggg

SEQ ID NO: 28997 - DNA, 28 bp, synthetic construct
  source 1..28: mol_type = other DNA
ttcacgtgtgtgtgtgggaccccttggg

SEQ ID NO: 28998 - DNA, 28 bp, synthetic construct
  source 1..28: mol_type = other DNA
cttcacgtgtgtgtgtgggaccccttgg

SEQ ID NO: 28999 - DNA, 28 bp, synthetic construct
  source 1..28: mol_type = other DNA
caaggggtcccacacacacacgtgaagg

SEQ ID NO: 29000 - DNA, 28 bp, synthetic construct
  source 1..28: mol_type = other DNA
aaggggtcccacacacacacgtgaaggg

SEQ ID NO: 29001 - DNA, 28 bp, synthetic construct
  source 1..28: mol_type = other DNA
aggggtcccacacacacacgtgaagggg

SEQ ID NO: 29002 - DNA, 28 bp, synthetic construct
  source 1..28: mol_type = other DNA
gagtgtccccttcacgtgtgtgtgtggg

SEQ ID NO: 29003 - DNA, 28 bp, synthetic construct
  source 1..28: mol_type = other DNA
ggagtgtccccttcacgtgtgtgtgtgg

SEQ ID NO: 29004 - DNA, 28 bp, synthetic construct
  source 1..28: mol_type = other DNA
gtgaaggggacactcccaacccatgagg

SEQ ID NO: 29005 - DNA, 28 bp, synthetic construct
  source 1..28: mol_type = other DNA
tgaaggggacactcccaacccatgaggg

SEQ ID NO: 29006 - DNA, 28 bp, synthetic construct
  source 1..28: mol_type = other DNA
ggagggtgtgtttccctcatgggttggg

SEQ ID NO: 29007 - DNA, 28 bp, synthetic construct
  source 1..28: mol_type = other DNA
tggagggtgtgtttccctcatgggttgg

SEQ ID NO: 29008 - DNA, 28 bp, synthetic construct
  source 1..28: mol_type = other DNA
aggatggagggtgtgtttccctcatggg

SEQ ID NO: 29009 - DNA, 28 bp, synthetic construct
  source 1..28: mol_type = other DNA
gaggatggagggtgtgtttccctcatgg

SEQ ID NO: 29010 - DNA, 28 bp, synthetic construct
  source 1..28: mol_type = other DNA
gggaaacacaccctccatcctcctttgg

SEQ ID NO: 29011 - DNA, 28 bp, synthetic construct
  source 1..28: mol_type = other DNA
tggggttgaaccaaaggaggatggaggg

SEQ ID NO: 29012 - DNA, 28 bp, synthetic construct
  source 1..28: mol_type = other DNA
ctggggttgaaccaaaggaggatggagg

SEQ ID NO: 29013 - DNA, 28 bp, synthetic construct
  source 1..28: mol_type = other DNA
aggctggggttgaaccaaaggaggatgg

SEQ ID NO: 29014 - DNA, 28 bp, synthetic construct
  source 1..28: mol_type = other DNA
tcggaggctggggttgaaccaaaggagg

SEQ ID NO: 29015 - DNA, 28 bp, synthetic construct
  source 1..28: mol_type = other DNA
ttctcggaggctggggttgaaccaaagg

SEQ ID NO: 29016 - DNA, 28 bp, synthetic construct
  source 1..28: mol_type = other DNA
tggttcaaccccagcctccgagaacagg

SEQ ID NO: 29017 - DNA, 28 bp, synthetic construct
  source 1..28: mol_type = other DNA
tgaaattacctgttctcggaggctgggg

SEQ ID NO: 29018 - DNA, 28 bp, synthetic construct
  source 1..28: mol_type = other DNA
atgaaattacctgttctcggaggctggg

SEQ ID NO: 29019 - DNA, 28 bp, synthetic construct
  source 1..28: mol_type = other DNA
tatgaaattacctgttctcggaggctgg

SEQ ID NO: 29020 - DNA, 28 bp, synthetic construct
  source 1..28: mol_type = other DNA
agcctccgagaacaggtaatttcatagg

SEQ ID NO: 29021 - DNA, 28 bp, synthetic construct
  source 1..28: mol_type = other DNA
ctcctatgaaattacctgttctcggagg

SEQ ID NO: 29022 - DNA, 28 bp, synthetic construct
  source 1..28: mol_type = other DNA
aagctcctatgaaattacctgttctcgg

SEQ ID NO: 29023 - DNA, 28 bp, synthetic construct
  source 1..28: mol_type = other DNA
agtgactataaaggtgacaagtttgtgg

SEQ ID NO: 29024 - DNA, 28 bp, synthetic construct
  source 1..28: mol_type = other DNA
cacctttatagtcacttgaagaagttgg

SEQ ID NO: 29025 - DNA, 28 bp, synthetic construct
  source 1..28: mol_type = other DNA
ttccaacttcttcaagtgactataaagg

SEQ ID NO: 29026 - DNA, 28 bp, synthetic construct
  source 1..28: mol_type = other DNA
agttggaaaaatacagtgaaagtcctgg

SEQ ID NO: 29027 - DNA, 28 bp, synthetic construct
  source 1..28: mol_type = other DNA
taggctacatctctgttgtagcaccagg

SEQ ID NO: 29028 - DNA, 28 bp, synthetic construct
  source 1..28: mol_type = other DNA
aacacatgtaaagcttatctggcatagg

SEQ ID NO: 29029 - DNA, 28 bp, synthetic construct
  source 1..28: mol_type = other DNA
tgaggtaacacatgtaaagcttatctgg

SEQ ID NO: 29030 - DNA, 28 bp, synthetic construct
  source 1..28: mol_type = other DNA
tgttacctcattagtcactcaacacagg

SEQ ID NO: 29031 - DNA, 28 bp, synthetic construct
  source 1..28: mol_type = other DNA
gttacctcattagtcactcaacacaggg

SEQ ID NO: 29032 - DNA, 28 bp, synthetic construct
  source 1..28: mol_type = other DNA
atcaccctgtgttgagtgactaatgagg

SEQ ID NO: 29033 - DNA, 28 bp, synthetic construct
  source 1..28: mol_type = other DNA
actcaacacagggtgatcatcttacagg

SEQ ID NO: 29034 - DNA, 28 bp, synthetic construct
  source 1..28: mol_type = other DNA
gatcatcttacaggaagagatactgagg

SEQ ID NO: 29035 - DNA, 28 bp, synthetic construct
  source 1..28: mol_type = other DNA
cttacaggaagagatactgaggcacagg

SEQ ID NO: 29036 - DNA, 28 bp, synthetic construct
  source 1..28: mol_type = other DNA
aggcacaggaatgtcaacttgcctaagg

SEQ ID NO: 29037 - DNA, 28 bp, synthetic construct
  source 1..28: mol_type = other DNA
acttgcctaaggtcacaaagctagaagg

SEQ ID NO: 29038 - DNA, 28 bp, synthetic construct
  source 1..28: mol_type = other DNA
ttgttccttctagctttgtgaccttagg

SEQ ID NO: 29039 - DNA, 28 bp, synthetic construct
  source 1..28: mol_type = other DNA
gtcacaaagctagaaggaacaaaatagg

SEQ ID NO: 29040 - DNA, 28 bp, synthetic construct
  source 1..28: mol_type = other DNA
tcacaaagctagaaggaacaaaataggg

SEQ ID NO: 29041 - DNA, 28 bp, synthetic construct
  source 1..28: mol_type = other DNA
aatagggcttcaaacccagtcattttgg

SEQ ID NO: 29042 - DNA, 28 bp, synthetic construct
  source 1..28: mol_type = other DNA
tcaaacccagtcattttggctccaaagg

SEQ ID NO: 29043 - DNA, 28 bp, synthetic construct
  source 1..28: mol_type = other DNA
catagcctttggagccaaaatgactggg

SEQ ID NO: 29044 - DNA, 28 bp, synthetic construct
  source 1..28: mol_type = other DNA
gcatagcctttggagccaaaatgactgg

SEQ ID NO: 29045 - DNA, 28 bp, synthetic construct
  source 1..28: mol_type = other DNA
agcacagtggttaaggcatagcctttgg

SEQ ID NO: 29046 - DNA, 28 bp, synthetic construct
  source 1..28: mol_type = other DNA
caggcggcgcttagcacagtggttaagg

SEQ ID NO: 29047 - DNA, 28 bp, synthetic construct
  source 1..28: mol_type = other DNA
gttaagcaggcggcgcttagcacagtgg

SEQ ID NO: 29048 - DNA, 28 bp, synthetic construct
  source 1..28: mol_type = other DNA
ctgtgctaagcgccgcctgcttaaccgg

SEQ ID NO: 29049 - DNA, 28 bp, synthetic construct
  source 1..28: mol_type = other DNA
tgtgctaagcgccgcctgcttaaccggg

SEQ ID NO: 29050 - DNA, 28 bp, synthetic construct
  source 1..28: mol_type = other DNA
ggaaaaggtagcccggttaagcaggcgg

SEQ ID NO: 29051 - DNA, 28 bp, synthetic construct
  source 1..28: mol_type = other DNA
ggtggaaaaggtagcccggttaagcagg

SEQ ID NO: 29052 - DNA, 28 bp, synthetic construct
  source 1..28: mol_type = other DNA
agaaattgtggtggaaaaggtagcccgg

SEQ ID NO: 29053 - DNA, 28 bp, synthetic construct
  source 1..28: mol_type = other DNA
aagggatgagaaattgtggtggaaaagg

SEQ ID NO: 29054 - DNA, 28 bp, synthetic construct
  source 1..28: mol_type = other DNA
tttcagaagggatgagaaattgtggtgg

SEQ ID NO: 29055 - DNA, 28 bp, synthetic construct
  source 1..28: mol_type = other DNA
atctttcagaagggatgagaaattgtgg

SEQ ID NO: 29056 - DNA, 28 bp, synthetic construct
  source 1..28: mol_type = other DNA
acaatttctcatcccttctgaaagatgg

SEQ ID NO: 29057 - DNA, 28 bp, synthetic construct
  source 1..28: mol_type = other DNA
ctcatcccttctgaaagatggtcacagg

SEQ ID NO: 29058 - DNA, 28 bp, synthetic construct
  source 1..28: mol_type = other DNA
caacacctgtgaccatctttcagaaggg

SEQ ID NO: 29059 - DNA, 28 bp, synthetic construct
  source 1..28: mol_type = other DNA
gcaacacctgtgaccatctttcagaagg

SEQ ID NO: 29060 - DNA, 28 bp, synthetic construct
  source 1..28: mol_type = other DNA
atggtcacaggtgttgctgaaatacagg

SEQ ID NO: 29061 - DNA, 28 bp, synthetic construct
  source 1..28: mol_type = other DNA
tagaattttaaatagttttacatttagg

SEQ ID NO: 29062 - DNA, 28 bp, synthetic construct
  source 1..28: mol_type = other DNA
agaattttaaatagttttacatttaggg

SEQ ID NO: 29063 - DNA, 28 bp, synthetic construct
  source 1..28: mol_type = other DNA
gaattttaaatagttttacatttagggg

SEQ ID NO: 29064 - DNA, 28 bp, synthetic construct
  source 1..28: mol_type = other DNA
gaacccttgtatacccctcaccccctgg

SEQ ID NO: 29065 - DNA, 28 bp, synthetic construct
  source 1..28: mol_type = other DNA
tatccagggggtgaggggtatacaaggg

SEQ ID NO: 29066 - DNA, 28 bp, synthetic construct
  source 1..28: mol_type = other DNA
gtatccagggggtgaggggtatacaagg

SEQ ID NO: 29067 - DNA, 28 bp, synthetic construct
  source 1..28: mol_type = other DNA
aagtgaggggtatccagggggtgagggg

SEQ ID NO: 29068 - DNA, 28 bp, synthetic construct
  source 1..28: mol_type = other DNA
caagtgaggggtatccagggggtgaggg

SEQ ID NO: 29069 - DNA, 28 bp, synthetic construct
  source 1..28: mol_type = other DNA
ccaagtgaggggtatccagggggtgagg

SEQ ID NO: 29070 - DNA, 28 bp, synthetic construct
  source 1..28: mol_type = other DNA
ataaaccaagtgaggggtatccaggggg

SEQ ID NO: 29071 - DNA, 28 bp, synthetic construct
  source 1..28: mol_type = other DNA
aataaaccaagtgaggggtatccagggg

SEQ ID NO: 29072 - DNA, 28 bp, synthetic construct
  source 1..28: mol_type = other DNA
gaataaaccaagtgaggggtatccaggg

SEQ ID NO: 29073 - DNA, 28 bp, synthetic construct
  source 1..28: mol_type = other DNA
agaataaaccaagtgaggggtatccagg

SEQ ID NO: 29074 - DNA, 28 bp, synthetic construct
  source 1..28: mol_type = other DNA
gtaacaacagaataaaccaagtgagggg

SEQ ID NO: 29075 - DNA, 28 bp, synthetic construct
  source 1..28: mol_type = other DNA
ggtaacaacagaataaaccaagtgaggg

SEQ ID NO: 29076 - DNA, 28 bp, synthetic construct
  source 1..28: mol_type = other DNA
tggtaacaacagaataaaccaagtgagg

SEQ ID NO: 29077 - DNA, 28 bp, synthetic construct
  source 1..28: mol_type = other DNA
tgacagatgtacgtagtaatgtcaatgg

SEQ ID NO: 29078 - DNA, 28 bp, synthetic construct
  source 1..28: mol_type = other DNA
attactacgtacatctgtcacaatgagg

SEQ ID NO: 29079 - DNA, 28 bp, synthetic construct
  source 1..28: mol_type = other DNA
ttactacgtacatctgtcacaatgaggg

SEQ ID NO: 29080 - DNA, 28 bp, synthetic construct
  source 1..28: mol_type = other DNA
ctacgtacatctgtcacaatgagggagg

SEQ ID NO: 29081 - DNA, 28 bp, synthetic construct
  source 1..28: mol_type = other DNA
tctgtcacaatgagggaggcaacactgg

SEQ ID NO: 29082 - DNA, 28 bp, synthetic construct
  source 1..28: mol_type = other DNA
tattgactacacgctacactttctttgg

SEQ ID NO: 29083 - DNA, 28 bp, synthetic construct
  source 1..28: mol_type = other DNA
tcttgggacagaaaaggacattaagggg

SEQ ID NO: 29084 - DNA, 28 bp, synthetic construct
  source 1..28: mol_type = other DNA
atcttgggacagaaaaggacattaaggg

SEQ ID NO: 29085 - DNA, 28 bp, synthetic construct
  source 1..28: mol_type = other DNA
gatcttgggacagaaaaggacattaagg

SEQ ID NO: 29086 - DNA, 28 bp, synthetic construct
  source 1..28: mol_type = other DNA
gtgggatgggatcttgggacagaaaagg

SEQ ID NO: 29087 - DNA, 28 bp, synthetic construct
  source 1..28: mol_type = other DNA
tctaaacgtagtgggatgggatcttggg

SEQ ID NO: 29088 - DNA, 28 bp, synthetic construct
  source 1..28: mol_type = other DNA
ctctaaacgtagtgggatgggatcttgg

SEQ ID NO: 29089 - DNA, 28 bp, synthetic construct
  source 1..28: mol_type = other DNA
ccatgagctctaaacgtagtgggatggg

SEQ ID NO: 29090 - DNA, 28 bp, synthetic construct
  source 1..28: mol_type = other DNA
gccatgagctctaaacgtagtgggatgg

SEQ ID NO: 29091 - DNA, 28 bp, synthetic construct
  source 1..28: mol_type = other DNA
aggagccatgagctctaaacgtagtggg

SEQ ID NO: 29092 - DNA, 28 bp, synthetic construct
  source 1..28: mol_type = other DNA
aaggagccatgagctctaaacgtagtgg

SEQ ID NO: 29093 - DNA, 28 bp, synthetic construct
  source 1..28: mol_type = other DNA
gtttagagctcatggctcctttgcctgg

SEQ ID NO: 29094 - DNA, 28 bp, synthetic construct
  source 1..28: mol_type = other DNA
gagctcatggctcctttgcctggcctgg

SEQ ID NO: 29095 - DNA, 28 bp, synthetic construct
  source 1..28: mol_type = other DNA
aagtgtcactgaccaggccaggcaaagg

SEQ ID NO: 29096 - DNA, 28 bp, synthetic construct
  source 1..28: mol_type = other DNA
tgagcaaagtgtcactgaccaggccagg

SEQ ID NO: 29097 - DNA, 28 bp, synthetic construct
  source 1..28: mol_type = other DNA
aagtctgagcaaagtgtcactgaccagg

SEQ ID NO: 29098 - DNA, 28 bp, synthetic construct
  source 1..28: mol_type = other DNA
cttcccttgttttcgatgacgttgatgg

SEQ ID NO: 29099 - DNA, 28 bp, synthetic construct
  source 1..28: mol_type = other DNA
agaccatcaacgtcatcgaaaacaaggg

SEQ ID NO: 29100 - DNA, 28 bp, synthetic construct
  source 1..28: mol_type = other DNA
aagaccatcaacgtcatcgaaaacaagg

SEQ ID NO: 29101 - DNA, 28 bp, synthetic construct
  source 1..28: mol_type = other DNA
gttttcgatgacgttgatggtcttgagg

SEQ ID NO: 29102 - DNA, 28 bp, synthetic construct
  source 1..28: mol_type = other DNA
gttgatggtcttgaggaacactgccagg

SEQ ID NO: 29103 - DNA, 28 bp, synthetic construct
  source 1..28: mol_type = other DNA
gtcttgaggaacactgccaggcatttgg

SEQ ID NO: 29104 - DNA, 28 bp, synthetic construct
  source 1..28: mol_type = other DNA
attgagggatattttaccaaatgcctgg

SEQ ID NO: 29105 - DNA, 28 bp, synthetic construct
  source 1..28: mol_type = other DNA
catttggtaaaatatccctcaatgtagg

SEQ ID NO: 29106 - DNA, 28 bp, synthetic construct
  source 1..28: mol_type = other DNA
aaagcatcagtcaaacctacattgaggg

SEQ ID NO: 29107 - DNA, 28 bp, synthetic construct
  source 1..28: mol_type = other DNA
aaaagcatcagtcaaacctacattgagg

SEQ ID NO: 29108 - DNA, 28 bp, synthetic construct
  source 1..28: mol_type = other DNA
ctcactcatcactagacccagattatgg

SEQ ID NO: 29109 - DNA, 28 bp, synthetic construct
  source 1..28: mol_type = other DNA
tcactcatcactagacccagattatggg

SEQ ID NO: 29110 - DNA, 28 bp, synthetic construct
  source 1..28: mol_type = other DNA
actagacccagattatgggtttttcagg

SEQ ID NO: 29111 - DNA, 28 bp, synthetic construct
  source 1..28: mol_type = other DNA
ctgtgacctgaaaaacccataatctggg

SEQ ID NO: 29112 - DNA, 28 bp, synthetic construct
  source 1..28: mol_type = other DNA
tctgtgacctgaaaaacccataatctgg

SEQ ID NO: 29113 - DNA, 28 bp, synthetic construct
  source 1..28: mol_type = other DNA
acatccttctcaccacatcctgtcaagg

SEQ ID NO: 29114 - DNA, 28 bp, synthetic construct
  source 1..28: mol_type = other DNA
cacaccttgacaggatgtggtgagaagg

SEQ ID NO: 29115 - DNA, 28 bp, synthetic construct
  source 1..28: mol_type = other DNA
gactatgtcacaccttgacaggatgtgg

SEQ ID NO: 29116 - DNA, 28 bp, synthetic construct
  source 1..28: mol_type = other DNA
cacatcgactatgtcacaccttgacagg

SEQ ID NO: 29117 - DNA, 28 bp, synthetic construct
  source 1..28: mol_type = other DNA
gacatagtcgatgtgaactgatcactgg

SEQ ID NO: 29118 - DNA, 28 bp, synthetic construct
  source 1..28: mol_type = other DNA
acatagtcgatgtgaactgatcactggg

SEQ ID NO: 29119 - DNA, 28 bp, synthetic construct
  source 1..28: mol_type = other DNA
tcactgggatgagaaactgtttgccagg

SEQ ID NO: 29120 - DNA, 28 bp, synthetic construct
  source 1..28: mol_type = other DNA
aaagtaacttagaggtggagaaacctgg

SEQ ID NO: 29121 - DNA, 28 bp, synthetic construct
  source 1..28: mol_type = other DNA
gcaaggaaagaaagtaacttagaggtgg

SEQ ID NO: 29122 - DNA, 28 bp, synthetic construct
  source 1..28: mol_type = other DNA
agggcaaggaaagaaagtaacttagagg

SEQ ID NO: 29123 - DNA, 28 bp, synthetic construct
  source 1..28: mol_type = other DNA
tagcttcaaacatcacactagggcaagg

SEQ ID NO: 29124 - DNA, 28 bp, synthetic construct
  source 1..28: mol_type = other DNA
ggacttagcttcaaacatcacactaggg

SEQ ID NO: 29125 - DNA, 28 bp, synthetic construct
  source 1..28: mol_type = other DNA
gggacttagcttcaaacatcacactagg

SEQ ID NO: 29126 - DNA, 28 bp, synthetic construct
  source 1..28: mol_type = other DNA
agtcccaaagtgcagcccatgctgtagg

SEQ ID NO: 29127 - DNA, 28 bp, synthetic construct
  source 1..28: mol_type = other DNA
attcctacagcatgggctgcactttggg

SEQ ID NO: 29128 - DNA, 28 bp, synthetic construct
  source 1..28: mol_type = other DNA
cattcctacagcatgggctgcactttgg

SEQ ID NO: 29129 - DNA, 28 bp, synthetic construct
  source 1..28: mol_type = other DNA
aagtgcagcccatgctgtaggaatgagg

SEQ ID NO: 29130 - DNA, 28 bp, synthetic construct
  source 1..28: mol_type = other DNA
gcttaactcctcattcctacagcatggg

SEQ ID NO: 29131 - DNA, 28 bp, synthetic construct
  source 1..28: mol_type = other DNA
agcttaactcctcattcctacagcatgg

SEQ ID NO: 29132 - DNA, 28 bp, synthetic construct
  source 1..28: mol_type = other DNA
gaggagttaagctccatctccttaatgg

SEQ ID NO: 29133 - DNA, 28 bp, synthetic construct
  source 1..28: mol_type = other DNA
aggagttaagctccatctccttaatggg

SEQ ID NO: 29134 - DNA, 28 bp, synthetic construct
  source 1..28: mol_type = other DNA
ggagttaagctccatctccttaatgggg

SEQ ID NO: 29135 - DNA, 28 bp, synthetic construct
  source 1..28: mol_type = other DNA
atatagttactccccattaaggagatgg

SEQ ID NO: 29136 - DNA, 28 bp, synthetic construct
  source 1..28: mol_type = other DNA
atatttatatagttactccccattaagg

SEQ ID NO: 29137 - DNA, 28 bp, synthetic construct
  source 1..28: mol_type = other DNA
ataaatataaccttatttttaatgatgg

SEQ ID NO: 29138 - DNA, 28 bp, synthetic construct
  source 1..28: mol_type = other DNA
tacggattaaccatcattaaaaataagg

SEQ ID NO: 29139 - DNA, 28 bp, synthetic construct
  source 1..28: mol_type = other DNA
tatttttaatgatggttaatccgtatgg

SEQ ID NO: 29140 - DNA, 28 bp, synthetic construct
  source 1..28: mol_type = other DNA
ttgttttattttttttaatgccatacgg

SEQ ID NO: 29141 - DNA, 28 bp, synthetic construct
  source 1..28: mol_type = other DNA
aaacaacatgccaagtgacagtgtacgg

SEQ ID NO: 29142 - DNA, 28 bp, synthetic construct
  source 1..28: mol_type = other DNA
tagggaagggccgtacactgtcacttgg

SEQ ID NO: 29143 - DNA, 28 bp, synthetic construct
  source 1..28: mol_type = other DNA
ctgcagagtcagcaacaatagggaaggg

SEQ ID NO: 29144 - DNA, 28 bp, synthetic construct
  source 1..28: mol_type = other DNA
actgcagagtcagcaacaatagggaagg

SEQ ID NO: 29145 - DNA, 28 bp, synthetic construct
  source 1..28: mol_type = other DNA
ttccctattgttgctgactctgcagtgg

SEQ ID NO: 29146 - DNA, 28 bp, synthetic construct
  source 1..28: mol_type = other DNA
agccactgcagagtcagcaacaataggg

SEQ ID NO: 29147 - DNA, 28 bp, synthetic construct
  source 1..28: mol_type = other DNA
cagccactgcagagtcagcaacaatagg

SEQ ID NO: 29148 - DNA, 28 bp, synthetic construct
  source 1..28: mol_type = other DNA
gttgctgactctgcagtggctgtaatgg

SEQ ID NO: 29149 - DNA, 28 bp, synthetic construct
  source 1..28: mol_type = other DNA
gtgattctgagacataaagatgatcagg

SEQ ID NO: 29150 - DNA, 28 bp, synthetic construct
  source 1..28: mol_type = other DNA
gatcatctttatgtctcagaatcacagg

SEQ ID NO: 29151 - DNA, 28 bp, synthetic construct
  source 1..28: mol_type = other DNA
catctttatgtctcagaatcacaggagg

SEQ ID NO: 29152 - DNA, 28 bp, synthetic construct
  source 1..28: mol_type = other DNA
caggaggtaagaagcactatctccaagg

SEQ ID NO: 29153 - DNA, 28 bp, synthetic construct
  source 1..28: mol_type = other DNA
cagttgttttacttttttgtcaccttgg

SEQ ID NO: 29154 - DNA, 28 bp, synthetic construct
  source 1..28: mol_type = other DNA
caaggtgacaaaaaagtaaaacaactgg

SEQ ID NO: 29155 - DNA, 28 bp, synthetic construct
  source 1..28: mol_type = other DNA
aaaaaagtaaaacaactggccagcatgg

SEQ ID NO: 29156 - DNA, 28 bp, synthetic construct
  source 1..28: mol_type = other DNA
taaaacaactggccagcatggaaagagg

SEQ ID NO: 29157 - DNA, 28 bp, synthetic construct
  source 1..28: mol_type = other DNA
aaaacaactggccagcatggaaagaggg

SEQ ID NO: 29158 - DNA, 28 bp, synthetic construct
  source 1..28: mol_type = other DNA
ggaatggacttccctctttccatgctgg

SEQ ID NO: 29159 - DNA, 28 bp, synthetic construct
  source 1..28: mol_type = other DNA
ttgttaaacatcatctagaatggaatgg

SEQ ID NO: 29160 - DNA, 28 bp, synthetic construct
  source 1..28: mol_type = other DNA
gttgtttgttaaacatcatctagaatgg

SEQ ID NO: 29161 - DNA, 28 bp, synthetic construct
  source 1..28: mol_type = other DNA
ttctagatgatgtttaacaaacaacagg

SEQ ID NO: 29162 - DNA, 28 bp, synthetic construct
  source 1..28: mol_type = other DNA
ttaacaaacaacaggagtcagagaaagg

SEQ ID NO: 29163 - DNA, 28 bp, synthetic construct
  source 1..28: mol_type = other DNA
gaaaggagaaaaaactatcccatgatgg

SEQ ID NO: 29164 - DNA, 28 bp, synthetic construct
  source 1..28: mol_type = other DNA
aggagaaaaaactatcccatgatggagg

SEQ ID NO: 29165 - DNA, 28 bp, synthetic construct
  source 1..28: mol_type = other DNA
atgcagcatgtgttgcctccatcatggg

SEQ ID NO: 29166 - DNA, 28 bp, synthetic construct
  source 1..28: mol_type = other DNA
catgcagcatgtgttgcctccatcatgg

SEQ ID NO: 29167 - DNA, 28 bp, synthetic construct
  source 1..28: mol_type = other DNA
aggcaacacatgctgcatgtttgtatgg

SEQ ID NO: 29168 - DNA, 28 bp, synthetic construct
  source 1..28: mol_type = other DNA
ggcaacacatgctgcatgtttgtatggg

SEQ ID NO: 29169 - DNA, 28 bp, synthetic construct
  source 1..28: mol_type = other DNA
acacatgctgcatgtttgtatgggcagg

SEQ ID NO: 29170 - DNA, 28 bp, synthetic construct
  source 1..28: mol_type = other DNA
atgtttgtatgggcaggtattaaactgg

SEQ ID NO: 29171 - DNA, 28 bp, synthetic construct
  source 1..28: mol_type = other DNA
ttggaaatttatatctgtcattgcttgg

SEQ ID NO: 29172 - DNA, 28 bp, synthetic construct
  source 1..28: mol_type = other DNA
atgacagatataaatttccaaagtgagg

SEQ ID NO: 29173 - DNA, 28 bp, synthetic construct
  source 1..28: mol_type = other DNA
atataaatttccaaagtgaggtgccagg

SEQ ID NO: 29174 - DNA, 28 bp, synthetic construct
  source 1..28: mol_type = other DNA
ctttggagagcctggcacctcactttgg

SEQ ID NO: 29175 - DNA, 28 bp, synthetic construct
  source 1..28: mol_type = other DNA
caaagtgaggtgccaggctctccaaagg

SEQ ID NO: 29176 - DNA, 28 bp, synthetic construct
  source 1..28: mol_type = other DNA
ctttgaaaagctcctttggagagcctgg

SEQ ID NO: 29177 - DNA, 28 bp, synthetic construct
  source 1..28: mol_type = other DNA
acacattaactttgaaaagctcctttgg

SEQ ID NO: 29178 - DNA, 28 bp, synthetic construct
  source 1..28: mol_type = other DNA
tctgtttctcactcagagtaggtcgggg

SEQ ID NO: 29179 - DNA, 28 bp, synthetic construct
  source 1..28: mol_type = other DNA
ttctgtttctcactcagagtaggtcggg

SEQ ID NO: 29180 - DNA, 28 bp, synthetic construct
  source 1..28: mol_type = other DNA
cttctgtttctcactcagagtaggtcgg

SEQ ID NO: 29181 - DNA, 28 bp, synthetic construct
  source 1..28: mol_type = other DNA
ttgacttctgtttctcactcagagtagg

SEQ ID NO: 29182 - DNA, 28 bp, synthetic construct
  source 1..28: mol_type = other DNA
caacagagaattttgtttttctttgagg

SEQ ID NO: 29183 - DNA, 28 bp, synthetic construct
  source 1..28: mol_type = other DNA
aacagagaattttgtttttctttgaggg

SEQ ID NO: 29184 - DNA, 28 bp, synthetic construct
  source 1..28: mol_type = other DNA
acagagaattttgtttttctttgagggg

SEQ ID NO: 29185 - DNA, 28 bp, synthetic construct
  source 1..28: mol_type = other DNA
cagagaattttgtttttctttgaggggg

SEQ ID NO: 29186 - DNA, 28 bp, synthetic construct
  source 1..28: mol_type = other DNA
atcccctccaccatcaccaaagagatgg

SEQ ID NO: 29187 - DNA, 28 bp, synthetic construct
  source 1..28: mol_type = other DNA
tcccctccaccatcaccaaagagatggg

SEQ ID NO: 29188 - DNA, 28 bp, synthetic construct
  source 1..28: mol_type = other DNA
acccatctctttggtgatggtggagggg

SEQ ID NO: 29189 - DNA, 28 bp, synthetic construct
  source 1..28: mol_type = other DNA
tacccatctctttggtgatggtggaggg

SEQ ID NO: 29190 - DNA, 28 bp, synthetic construct
  source 1..28: mol_type = other DNA
ctacccatctctttggtgatggtggagg

SEQ ID NO: 29191 - DNA, 28 bp, synthetic construct
  source 1..28: mol_type = other DNA
gtgctacccatctctttggtgatggtgg

SEQ ID NO: 29192 - DNA, 28 bp, synthetic construct
  source 1..28: mol_type = other DNA
actgtgctacccatctctttggtgatgg

SEQ ID NO: 29193 - DNA, 28 bp, synthetic construct
  source 1..28: mol_type = other DNA
atcaccaaagagatgggtagcacagtgg

SEQ ID NO: 29194 - DNA, 28 bp, synthetic construct
  source 1..28: mol_type = other DNA
accaaagagatgggtagcacagtggagg

SEQ ID NO: 29195 - DNA, 28 bp, synthetic construct
  source 1..28: mol_type = other DNA
ccaaagagatgggtagcacagtggaggg

SEQ ID NO: 29196 - DNA, 28 bp, synthetic construct
  source 1..28: mol_type = other DNA
caaagagatgggtagcacagtggagggg

SEQ ID NO: 29197 - DNA, 28 bp, synthetic construct
  source 1..28: mol_type = other DNA
aaagagatgggtagcacagtggaggggg

SEQ ID NO: 29198 - DNA, 28 bp, synthetic construct
  source 1..28: mol_type = other DNA
aagagatgggtagcacagtggagggggg

SEQ ID NO: 29199 - DNA, 28 bp, synthetic construct
  source 1..28: mol_type = other DNA
agagatgggtagcacagtggaggggggg

SEQ ID NO: 29200 - DNA, 28 bp, synthetic construct
  source 1..28: mol_type = other DNA
gagatgggtagcacagtggagggggggg

SEQ ID NO: 29201 - DNA, 28 bp, synthetic construct
  source 1..28: mol_type = other DNA
agatgggtagcacagtggaggggggggg

SEQ ID NO: 29202 - DNA, 28 bp, synthetic construct
  source 1..28: mol_type = other DNA
gatgggtagcacagtggagggggggggg

SEQ ID NO: 29203 - DNA, 28 bp, synthetic construct
  source 1..28: mol_type = other DNA
atgggtagcacagtggaggggggggggg

SEQ ID NO: 29204 - DNA, 28 bp, synthetic construct
  source 1..28: mol_type = other DNA
tgccgactctcaagtccactgacagagg

SEQ ID NO: 29205 - DNA, 28 bp, synthetic construct
  source 1..28: mol_type = other DNA
agcctctgtcagtggacttgagagtcgg

SEQ ID NO: 29206 - DNA, 28 bp, synthetic construct
  source 1..28: mol_type = other DNA
atttctgctttgaagcctctgtcagtgg

SEQ ID NO: 29207 - DNA, 28 bp, synthetic construct
  source 1..28: mol_type = other DNA
acttgatataatttccgtagaattttgg

SEQ ID NO: 29208 - DNA, 28 bp, synthetic construct
  source 1..28: mol_type = other DNA
tgatataatttccgtagaattttggagg

SEQ ID NO: 29209 - DNA, 28 bp, synthetic construct
  source 1..28: mol_type = other DNA
tttccgtagaattttggaggcctgctgg

SEQ ID NO: 29210 - DNA, 28 bp, synthetic construct
  source 1..28: mol_type = other DNA
agtccagcaggcctccaaaattctacgg

SEQ ID NO: 29211 - DNA, 28 bp, synthetic construct
  source 1..28: mol_type = other DNA
gtagaattttggaggcctgctggactgg

SEQ ID NO: 29212 - DNA, 28 bp, synthetic construct
  source 1..28: mol_type = other DNA
tttggaggcctgctggactggcagctgg

SEQ ID NO: 29213 - DNA, 28 bp, synthetic construct
  source 1..28: mol_type = other DNA
gctgtgtaccagctgccagtccagcagg

SEQ ID NO: 29214 - DNA, 28 bp, synthetic construct
  source 1..28: mol_type = other DNA
cagctggtacacagctaaaagatagagg

SEQ ID NO: 29215 - DNA, 28 bp, synthetic construct
  source 1..28: mol_type = other DNA
agatagaggctagctaaaattgcactgg

SEQ ID NO: 29216 - DNA, 28 bp, synthetic construct
  source 1..28: mol_type = other DNA
gatagaggctagctaaaattgcactggg

SEQ ID NO: 29217 - DNA, 28 bp, synthetic construct
  source 1..28: mol_type = other DNA
gaggctagctaaaattgcactgggaagg

SEQ ID NO: 29218 - DNA, 28 bp, synthetic construct
  source 1..28: mol_type = other DNA
ccacttcagagggagaatgcagttcagg

SEQ ID NO: 29219 - DNA, 28 bp, synthetic construct
  source 1..28: mol_type = other DNA
gaactgcattctccctctgaagtggagg

SEQ ID NO: 29220 - DNA, 28 bp, synthetic construct
  source 1..28: mol_type = other DNA
gcattctccctctgaagtggaggaaagg

SEQ ID NO: 29221 - DNA, 28 bp, synthetic construct
  source 1..28: mol_type = other DNA
taaggtgcctttcctccacttcagaggg

SEQ ID NO: 29222 - DNA, 28 bp, synthetic construct
  source 1..28: mol_type = other DNA
ttaaggtgcctttcctccacttcagagg

SEQ ID NO: 29223 - DNA, 28 bp, synthetic construct
  source 1..28: mol_type = other DNA
gaagtggaggaaaggcaccttaatttgg

SEQ ID NO: 29224 - DNA, 28 bp, synthetic construct
  source 1..28: mol_type = other DNA
aagtggaggaaaggcaccttaatttggg

SEQ ID NO: 29225 - DNA, 28 bp, synthetic construct
  source 1..28: mol_type = other DNA
attctacatctggcttcccaaattaagg

SEQ ID NO: 29226 - DNA, 28 bp, synthetic construct
  source 1..28: mol_type = other DNA
gggaagccagatgtagaatttatgatgg

SEQ ID NO: 29227 - DNA, 28 bp, synthetic construct
  source 1..28: mol_type = other DNA
ggaagccagatgtagaatttatgatggg

SEQ ID NO: 29228 - DNA, 28 bp, synthetic construct
  source 1..28: mol_type = other DNA
gaagccagatgtagaatttatgatgggg

SEQ ID NO: 29229 - DNA, 28 bp, synthetic construct
  source 1..28: mol_type = other DNA
acatccccatcataaattctacatctgg

SEQ ID NO: 29230 - DNA, 28 bp, synthetic construct
  source 1..28: mol_type = other DNA
gaatttatgatggggatgtcgaccaagg

SEQ ID NO: 29231 - DNA, 28 bp, synthetic construct
  source 1..28: mol_type = other DNA
agaaatctcttgggcaggatgaccttgg

SEQ ID NO: 29232 - DNA, 28 bp, synthetic construct
  source 1..28: mol_type = other DNA
tcatcctgcccaagagatttcttccagg

SEQ ID NO: 29233 - DNA, 28 bp, synthetic construct
  source 1..28: mol_type = other DNA
catcctgcccaagagatttcttccaggg

SEQ ID NO: 29234 - DNA, 28 bp, synthetic construct
  source 1..28: mol_type = other DNA
atcctgcccaagagatttcttccagggg

SEQ ID NO: 29235 - DNA, 28 bp, synthetic construct
  source 1..28: mol_type = other DNA
tcctgcccaagagatttcttccaggggg

SEQ ID NO: 29236 - DNA, 28 bp, synthetic construct
  source 1..28: mol_type = other DNA
accccctggaagaaatctcttgggcagg

SEQ ID NO: 29237 - DNA, 28 bp, synthetic construct
  source 1..28: mol_type = other DNA
tctgaccccctggaagaaatctcttggg

SEQ ID NO: 29238 - DNA, 28 bp, synthetic construct
  source 1..28: mol_type = other DNA
atctgaccccctggaagaaatctcttgg

SEQ ID NO: 29239 - DNA, 28 bp, synthetic construct
  source 1..28: mol_type = other DNA
aagagatttcttccagggggtcagatgg

SEQ ID NO: 29240 - DNA, 28 bp, synthetic construct
  source 1..28: mol_type = other DNA
ttccagggggtcagatggacccagcagg

SEQ ID NO: 29241 - DNA, 28 bp, synthetic construct
  source 1..28: mol_type = other DNA
tccagggggtcagatggacccagcaggg

SEQ ID NO: 29242 - DNA, 28 bp, synthetic construct
  source 1..28: mol_type = other DNA
accctgctgggtccatctgaccccctgg

SEQ ID NO: 29243 - DNA, 28 bp, synthetic construct
  source 1..28: mol_type = other DNA
ggggtcagatggacccagcagggtctgg

SEQ ID NO: 29244 - DNA, 28 bp, synthetic construct
  source 1..28: mol_type = other DNA
agatggacccagcagggtctggatgagg

SEQ ID NO: 29245 - DNA, 28 bp, synthetic construct
  source 1..28: mol_type = other DNA
agatctgcctcatccagaccctgctggg

SEQ ID NO: 29246 - DNA, 28 bp, synthetic construct
  source 1..28: mol_type = other DNA
gagatctgcctcatccagaccctgctgg

SEQ ID NO: 29247 - DNA, 28 bp, synthetic construct
  source 1..28: mol_type = other DNA
ataaaatcagaagctgcgagcaatgtgg

SEQ ID NO: 29248 - DNA, 28 bp, synthetic construct
  source 1..28: mol_type = other DNA
taaaatcagaagctgcgagcaatgtggg

SEQ ID NO: 29249 - DNA, 28 bp, synthetic construct
  source 1..28: mol_type = other DNA
agaagctgcgagcaatgtgggagcaagg

SEQ ID NO: 29250 - DNA, 28 bp, synthetic construct
  source 1..28: mol_type = other DNA
gaagctgcgagcaatgtgggagcaaggg

SEQ ID NO: 29251 - DNA, 28 bp, synthetic construct
  source 1..28: mol_type = other DNA
ctgcgagcaatgtgggagcaagggaagg

SEQ ID NO: 29252 - DNA, 28 bp, synthetic construct
  source 1..28: mol_type = other DNA
agcaatgtgggagcaagggaaggcaagg

SEQ ID NO: 29253 - DNA, 28 bp, synthetic construct
  source 1..28: mol_type = other DNA
aagggaaggcaaggctgccagagtaagg

SEQ ID NO: 29254 - DNA, 28 bp, synthetic construct
  source 1..28: mol_type = other DNA
ggaaggcaaggctgccagagtaaggtgg

SEQ ID NO: 29255 - DNA, 28 bp, synthetic construct
  source 1..28: mol_type = other DNA
gctgccagagtaaggtggctgcagttgg

SEQ ID NO: 29256 - DNA, 28 bp, synthetic construct
  source 1..28: mol_type = other DNA
gccagagtaaggtggctgcagttggagg

SEQ ID NO: 29257 - DNA, 28 bp, synthetic construct
  source 1..28: mol_type = other DNA
ccagagtaaggtggctgcagttggaggg

SEQ ID NO: 29258 - DNA, 28 bp, synthetic construct
  source 1..28: mol_type = other DNA
cagagtaaggtggctgcagttggagggg

SEQ ID NO: 29259 - DNA, 28 bp, synthetic construct
  source 1..28: mol_type = other DNA
ggctgcagttggaggggcccagcagagg

SEQ ID NO: 29260 - DNA, 28 bp, synthetic construct
  source 1..28: mol_type = other DNA
tggaggggcccagcagaggagcacacgg

SEQ ID NO: 29261 - DNA, 28 bp, synthetic construct
  source 1..28: mol_type = other DNA
tgggcactccgtgtgctcctctgctggg

SEQ ID NO: 29262 - DNA, 28 bp, synthetic construct
  source 1..28: mol_type = other DNA
atgggcactccgtgtgctcctctgctgg

SEQ ID NO: 29263 - DNA, 28 bp, synthetic construct
  source 1..28: mol_type = other DNA
cagaggagcacacggagtgcccatgtgg

SEQ ID NO: 29264 - DNA, 28 bp, synthetic construct
  source 1..28: mol_type = other DNA
ggagcacacggagtgcccatgtggaagg

SEQ ID NO: 29265 - DNA, 28 bp, synthetic construct
  source 1..28: mol_type = other DNA
gctggttttaaagggccttccacatggg

SEQ ID NO: 29266 - DNA, 28 bp, synthetic construct
  source 1..28: mol_type = other DNA
agctggttttaaagggccttccacatgg

SEQ ID NO: 29267 - DNA, 28 bp, synthetic construct
  source 1..28: mol_type = other DNA
gtggaaggccctttaaaaccagctcagg

SEQ ID NO: 29268 - DNA, 28 bp, synthetic construct
  source 1..28: mol_type = other DNA
tctggaagcctgagctggttttaaaggg

SEQ ID NO: 29269 - DNA, 28 bp, synthetic construct
  source 1..28: mol_type = other DNA
ttctggaagcctgagctggttttaaagg

SEQ ID NO: 29270 - DNA, 28 bp, synthetic construct
  source 1..28: mol_type = other DNA
aaaccagctcaggcttccagaagtatgg

SEQ ID NO: 29271 - DNA, 28 bp, synthetic construct
  source 1..28: mol_type = other DNA
ctgccatacttctggaagcctgagctgg

SEQ ID NO: 29272 - DNA, 28 bp, synthetic construct
  source 1..28: mol_type = other DNA
caagagtattagtctgccatacttctgg

SEQ ID NO: 29273 - DNA, 28 bp, synthetic construct
  source 1..28: mol_type = other DNA
taattggttttcattcattcattactgg

SEQ ID NO: 29274 - DNA, 28 bp, synthetic construct
  source 1..28: mol_type = other DNA
tgaaaaccaattattattgttttgttgg

SEQ ID NO: 29275 - DNA, 28 bp, synthetic construct
  source 1..28: mol_type = other DNA
gaaaaccaattattattgttttgttggg

SEQ ID NO: 29276 - DNA, 28 bp, synthetic construct
  source 1..28: mol_type = other DNA
ctgaacccaacaaaacaataataattgg

SEQ ID NO: 29277 - DNA, 28 bp, synthetic construct
  source 1..28: mol_type = other DNA
attattattgttttgttgggttcagagg

SEQ ID NO: 29278 - DNA, 28 bp, synthetic construct
  source 1..28: mol_type = other DNA
gaggaaatgaaaaaaaaatgtctacagg

SEQ ID NO: 29279 - DNA, 28 bp, synthetic construct
  source 1..28: mol_type = other DNA
aggaaatgaaaaaaaaatgtctacaggg

SEQ ID NO: 29280 - DNA, 28 bp, synthetic construct
  source 1..28: mol_type = other DNA
ggaaatgaaaaaaaaatgtctacagggg

SEQ ID NO: 29281 - DNA, 28 bp, synthetic construct
  source 1..28: mol_type = other DNA
aaaaaaaatgtctacaggggcaaaaagg

SEQ ID NO: 29282 - DNA, 28 bp, synthetic construct
  source 1..28: mol_type = other DNA
aatgtctacaggggcaaaaaggaaaagg

SEQ ID NO: 29283 - DNA, 28 bp, synthetic construct
  source 1..28: mol_type = other DNA
acaaacagtaacaaccaaaaatccctgg

SEQ ID NO: 29284 - DNA, 28 bp, synthetic construct
  source 1..28: mol_type = other DNA
caaacagtaacaaccaaaaatccctggg

SEQ ID NO: 29285 - DNA, 28 bp, synthetic construct
  source 1..28: mol_type = other DNA
ctgaggctcactgcccagggatttttgg

SEQ ID NO: 29286 - DNA, 28 bp, synthetic construct
  source 1..28: mol_type = other DNA
atccctgggcagtgagcctcagaaaagg

SEQ ID NO: 29287 - DNA, 28 bp, synthetic construct
  source 1..28: mol_type = other DNA
tccctgggcagtgagcctcagaaaaggg

SEQ ID NO: 29288 - DNA, 28 bp, synthetic construct
  source 1..28: mol_type = other DNA
ccccttttctgaggctcactgcccaggg

SEQ ID NO: 29289 - DNA, 28 bp, synthetic construct
  source 1..28: mol_type = other DNA
tccccttttctgaggctcactgcccagg

SEQ ID NO: 29290 - DNA, 28 bp, synthetic construct
  source 1..28: mol_type = other DNA
ggcagtgagcctcagaaaaggggaacgg

SEQ ID NO: 29291 - DNA, 28 bp, synthetic construct
  source 1..28: mol_type = other DNA
ctcacaggaccgttccccttttctgagg

SEQ ID NO: 29292 - DNA, 28 bp, synthetic construct
  source 1..28: mol_type = other DNA
ctcagaaaaggggaacggtcctgtgagg

SEQ ID NO: 29293 - DNA, 28 bp, synthetic construct
  source 1..28: mol_type = other DNA
aggggaacggtcctgtgaggacatgtgg

SEQ ID NO: 29294 - DNA, 28 bp, synthetic construct
  source 1..28: mol_type = other DNA
acgtgagatcaccacatgtcctcacagg

SEQ ID NO: 29295 - DNA, 28 bp, synthetic construct
  source 1..28: mol_type = other DNA
acatgtggtgatctcacgtgatctctgg

SEQ ID NO: 29296 - DNA, 28 bp, synthetic construct
  source 1..28: mol_type = other DNA
catgtggtgatctcacgtgatctctggg

SEQ ID NO: 29297 - DNA, 28 bp, synthetic construct
  source 1..28: mol_type = other DNA
gtggtgatctcacgtgatctctgggagg

SEQ ID NO: 29298 - DNA, 28 bp, synthetic construct
  source 1..28: mol_type = other DNA
tgatctcacgtgatctctgggaggctgg

SEQ ID NO: 29299 - DNA, 28 bp, synthetic construct
  source 1..28: mol_type = other DNA
gatctcacgtgatctctgggaggctggg

SEQ ID NO: 29300 - DNA, 28 bp, synthetic construct
  source 1..28: mol_type = other DNA
tctgggaggctgggcctcagctctgtgg

SEQ ID NO: 29301 - DNA, 28 bp, synthetic construct
  source 1..28: mol_type = other DNA
ggaggctgggcctcagctctgtggctgg

SEQ ID NO: 29302 - DNA, 28 bp, synthetic construct
  source 1..28: mol_type = other DNA
gaggctgggcctcagctctgtggctggg

SEQ ID NO: 29303 - DNA, 28 bp, synthetic construct
  source 1..28: mol_type = other DNA
gctgggcctcagctctgtggctgggtgg

SEQ ID NO: 29304 - DNA, 28 bp, synthetic construct
  source 1..28: mol_type = other DNA
ctgggcctcagctctgtggctgggtggg

SEQ ID NO: 29305 - DNA, 28 bp, synthetic construct
  source 1..28: mol_type = other DNA
tgggcctcagctctgtggctgggtgggg

SEQ ID NO: 29306 - DNA, 28 bp, synthetic construct
  source 1..28: mol_type = other DNA
gggcctcagctctgtggctgggtggggg

SEQ ID NO: 29307 - DNA, 28 bp, synthetic construct
  source 1..28: mol_type = other DNA
gttcccccacccagccacagagctgagg

SEQ ID NO: 29308 - DNA, 28 bp, synthetic construct
  source 1..28: mol_type = other DNA
gggtgggggaactaaactaaaattccgg

SEQ ID NO: 29309 - DNA, 28 bp, synthetic construct
  source 1..28: mol_type = other DNA
ggtgggggaactaaactaaaattccggg

SEQ ID NO: 29310 - DNA, 28 bp, synthetic construct
  source 1..28: mol_type = other DNA
gtgggggaactaaactaaaattccgggg

SEQ ID NO: 29311 - DNA, 28 bp, synthetic construct
  source 1..28: mol_type = other DNA
actaaactaaaattccggggttacatgg

SEQ ID NO: 29312 - DNA, 28 bp, synthetic construct
  source 1..28: mol_type = other DNA
aattccggggttacatggcagcatctgg

SEQ ID NO: 29313 - DNA, 28 bp, synthetic construct
  source 1..28: mol_type = other DNA
ccttccagatgctgccatgtaaccccgg

SEQ ID NO: 29314 - DNA, 28 bp, synthetic construct
  source 1..28: mol_type = other DNA
ttacatggcagcatctggaaggcaatgg

SEQ ID NO: 29315 - DNA, 28 bp, synthetic construct
  source 1..28: mol_type = other DNA
atctggaaggcaatggaattgtctcagg

SEQ ID NO: 29316 - DNA, 28 bp, synthetic construct
  source 1..28: mol_type = other DNA
tgtctcaggaccgcagtacccccgcagg

SEQ ID NO: 29317 - DNA, 28 bp, synthetic construct
  source 1..28: mol_type = other DNA
gtgctgctgtcctgcgggggtactgcgg

SEQ ID NO: 29318 - DNA, 28 bp, synthetic construct
  source 1..28: mol_type = other DNA
gtcatagggtgctgctgtcctgcggggg

SEQ ID NO: 29319 - DNA, 28 bp, synthetic construct
  source 1..28: mol_type = other DNA
agtcatagggtgctgctgtcctgcgggg

SEQ ID NO: 29320 - DNA, 28 bp, synthetic construct
  source 1..28: mol_type = other DNA
tagtcatagggtgctgctgtcctgcggg

SEQ ID NO: 29321 - DNA, 28 bp, synthetic construct
  source 1..28: mol_type = other DNA
gtagtcatagggtgctgctgtcctgcgg

SEQ ID NO: 29322 - DNA, 28 bp, synthetic construct
  source 1..28: mol_type = other DNA
caggacagcagcaccctatgactactgg

SEQ ID NO: 29323 - DNA, 28 bp, synthetic construct
  source 1..28: mol_type = other DNA
gcttttgcttttgccagtagtcataggg

SEQ ID NO: 29324 - DNA, 28 bp, synthetic construct
  source 1..28: mol_type = other DNA
tgcttttgcttttgccagtagtcatagg

SEQ ID NO: 29325 - DNA, 28 bp, synthetic construct
  source 1..28: mol_type = other DNA
actctgagaaaagcatccttgacttagg

SEQ ID NO: 29326 - DNA, 28 bp, synthetic construct
  source 1..28: mol_type = other DNA
agaaaaagtcttggggcctaagtcaagg

SEQ ID NO: 29327 - DNA, 28 bp, synthetic construct
  source 1..28: mol_type = other DNA
aggccccaagactttttctacaattagg

SEQ ID NO: 29328 - DNA, 28 bp, synthetic construct
  source 1..28: mol_type = other DNA
gatcctaattgtagaaaaagtcttgggg

SEQ ID NO: 29329 - DNA, 28 bp, synthetic construct
  source 1..28: mol_type = other DNA
tgatcctaattgtagaaaaagtcttggg

SEQ ID NO: 29330 - DNA, 28 bp, synthetic construct
  source 1..28: mol_type = other DNA
ttgatcctaattgtagaaaaagtcttgg

SEQ ID NO: 29331 - DNA, 28 bp, synthetic construct
  source 1..28: mol_type = other DNA
tcaaccaaatatgagctagcaattaagg

SEQ ID NO: 29332 - DNA, 28 bp, synthetic construct
  source 1..28: mol_type = other DNA
taaaccttaattgctagctcatatttgg

SEQ ID NO: 29333 - DNA, 28 bp, synthetic construct
  source 1..28: mol_type = other DNA
agcaattaaggtttactaaacagacagg

SEQ ID NO: 29334 - DNA, 28 bp, synthetic construct
  source 1..28: mol_type = other DNA
gcaattaaggtttactaaacagacaggg

SEQ ID NO: 29335 - DNA, 28 bp, synthetic construct
  source 1..28: mol_type = other DNA
taaacagacagggaaacgaaacatcagg

SEQ ID NO: 29336 - DNA, 28 bp, synthetic construct
  source 1..28: mol_type = other DNA
gagaaagaacagatgcaaagtgccaagg

SEQ ID NO: 29337 - DNA, 28 bp, synthetic construct
  source 1..28: mol_type = other DNA
tggtaactgaagcatctgaagtccttgg

SEQ ID NO: 29338 - DNA, 28 bp, synthetic construct
  source 1..28: mol_type = other DNA
atgtagttattttatagtcagtatttgg

SEQ ID NO: 29339 - DNA, 28 bp, synthetic construct
  source 1..28: mol_type = other DNA
tgactataaaataactacatatgaaagg

SEQ ID NO: 29340 - DNA, 28 bp, synthetic construct
  source 1..28: mol_type = other DNA
taacaagtgactatcaaaaatgaccagg

SEQ ID NO: 29341 - DNA, 28 bp, synthetic construct
  source 1..28: mol_type = other DNA
aagtgactatcaaaaatgaccaggcagg

SEQ ID NO: 29342 - DNA, 28 bp, synthetic construct
  source 1..28: mol_type = other DNA
agtgactatcaaaaatgaccaggcaggg

SEQ ID NO: 29343 - DNA, 28 bp, synthetic construct
  source 1..28: mol_type = other DNA
actatcaaaaatgaccaggcagggctgg

SEQ ID NO: 29344 - DNA, 28 bp, synthetic construct
  source 1..28: mol_type = other DNA
ctatcaaaaatgaccaggcagggctggg

SEQ ID NO: 29345 - DNA, 28 bp, synthetic construct
  source 1..28: mol_type = other DNA
aatgaccaggcagggctgggtgcagtgg

SEQ ID NO: 29346 - DNA, 28 bp, synthetic construct
  source 1..28: mol_type = other DNA
gtgagccactgcacccagccctgcctgg

SEQ ID NO: 29347 - DNA, 28 bp, synthetic construct
  source 1..28: mol_type = other DNA
gctcacgaccgtaatcccaccactttgg

SEQ ID NO: 29348 - DNA, 28 bp, synthetic construct
  source 1..28: mol_type = other DNA
ctcacgaccgtaatcccaccactttggg

SEQ ID NO: 29349 - DNA, 28 bp, synthetic construct
  source 1..28: mol_type = other DNA
acgaccgtaatcccaccactttgggagg

SEQ ID NO: 29350 - DNA, 28 bp, synthetic construct
  source 1..28: mol_type = other DNA
ttggcctcccaaagtggtgggattacgg

SEQ ID NO: 29351 - DNA, 28 bp, synthetic construct
  source 1..28: mol_type = other DNA
gtaatcccaccactttgggaggccaagg

SEQ ID NO: 29352 - DNA, 28 bp, synthetic construct
  source 1..28: mol_type = other DNA
atcccaccactttgggaggccaaggcgg

SEQ ID NO: 29353 - DNA, 28 bp, synthetic construct
  source 1..28: mol_type = other DNA
tcccaccactttgggaggccaaggcggg

SEQ ID NO: 29354 - DNA, 28 bp, synthetic construct
  source 1..28: mol_type = other DNA
acccgccttggcctcccaaagtggtggg

SEQ ID NO: 29355 - DNA, 28 bp, synthetic construct
  source 1..28: mol_type = other DNA
cacccgccttggcctcccaaagtggtgg

SEQ ID NO: 29356 - DNA, 28 bp, synthetic construct
  source 1..28: mol_type = other DNA
caccactttgggaggccaaggcgggtgg

SEQ ID NO: 29357 - DNA, 28 bp, synthetic construct
  source 1..28: mol_type = other DNA
atccacccgccttggcctcccaaagtgg

SEQ ID NO: 29358 - DNA, 28 bp, synthetic construct
  source 1..28: mol_type = other DNA
ctggactcaggtgatccacccgccttgg

SEQ ID NO: 29359 - DNA, 28 bp, synthetic construct
  source 1..28: mol_type = other DNA
caaggcgggtggatcacctgagtccagg

SEQ ID NO: 29360 - DNA, 28 bp, synthetic construct
  source 1..28: mol_type = other DNA
gtggatcacctgagtccaggagttcagg

SEQ ID NO: 29361 - DNA, 28 bp, synthetic construct
  source 1..28: mol_type = other DNA
aggctggtcctgaactcctggactcagg

SEQ ID NO: 29362 - DNA, 28 bp, synthetic construct
  source 1..28: mol_type = other DNA
tgagtccaggagttcaggaccagcctgg

SEQ ID NO: 29363 - DNA, 28 bp, synthetic construct
  source 1..28: mol_type = other DNA
gttggccaggctggtcctgaactcctgg

SEQ ID NO: 29364 - DNA, 28 bp, synthetic construct
  source 1..28: mol_type = other DNA
gagttcaggaccagcctggccaacatgg

SEQ ID NO: 29365 - DNA, 28 bp, synthetic construct
  source 1..28: mol_type = other DNA
cggggtttcaccatgttggccaggctgg

SEQ ID NO: 29366 - DNA, 28 bp, synthetic construct
  source 1..28: mol_type = other DNA
gagacggggtttcaccatgttggccagg

SEQ ID NO: 29367 - DNA, 28 bp, synthetic construct
  source 1..28: mol_type = other DNA
tagtagagacggggtttcaccatgttgg

SEQ ID NO: 29368 - DNA, 28 bp, synthetic construct
  source 1..28: mol_type = other DNA
aatttttgtatttttagtagagacgggg

SEQ ID NO: 29369 - DNA, 28 bp, synthetic construct
  source 1..28: mol_type = other DNA
taatttttgtatttttagtagagacggg

SEQ ID NO: 29370 - DNA, 28 bp, synthetic construct
  source 1..28: mol_type = other DNA
ctaatttttgtatttttagtagagacgg

SEQ ID NO: 29371 - DNA, 28 bp, synthetic construct
  source 1..28: mol_type = other DNA
tctactaaaaatacaaaaattagccagg

SEQ ID NO: 29372 - DNA, 28 bp, synthetic construct
  source 1..28: mol_type = other DNA
taaaaatacaaaaattagccaggcgtgg

SEQ ID NO: 29373 - DNA, 28 bp, synthetic construct
  source 1..28: mol_type = other DNA
aaatacaaaaattagccaggcgtggtgg

SEQ ID NO: 29374 - DNA, 28 bp, synthetic construct
  source 1..28: mol_type = other DNA
gattacaggcaagtgccaccacgcctgg

SEQ ID NO: 29375 - DNA, 28 bp, synthetic construct
  source 1..28: mol_type = other DNA
cgtggtggcacttgcctgtaatcccagg

SEQ ID NO: 29376 - DNA, 28 bp, synthetic construct
  source 1..28: mol_type = other DNA
gcacttgcctgtaatcccaggtactcgg

SEQ ID NO: 29377 - DNA, 28 bp, synthetic construct
  source 1..28: mol_type = other DNA
cacttgcctgtaatcccaggtactcggg

SEQ ID NO: 29378 - DNA, 28 bp, synthetic construct
  source 1..28: mol_type = other DNA
ttgcctgtaatcccaggtactcgggagg

SEQ ID NO: 29379 - DNA, 28 bp, synthetic construct
  source 1..28: mol_type = other DNA
cagcctcccgagtacctgggattacagg

SEQ ID NO: 29380 - DNA, 28 bp, synthetic construct
  source 1..28: mol_type = other DNA
gtaatcccaggtactcgggaggctgagg

SEQ ID NO: 29381 - DNA, 28 bp, synthetic construct
  source 1..28: mol_type = other DNA
tcccaggtactcgggaggctgaggcagg

SEQ ID NO: 29382 - DNA, 28 bp, synthetic construct
  source 1..28: mol_type = other DNA
tcctgcctcagcctcccgagtacctggg

SEQ ID NO: 29383 - DNA, 28 bp, synthetic construct
  source 1..28: mol_type = other DNA
ctcctgcctcagcctcccgagtacctgg

SEQ ID NO: 29384 - DNA, 28 bp, synthetic construct
  source 1..28: mol_type = other DNA
ctgaggcaggagaatcacttgaacctgg

SEQ ID NO: 29385 - DNA, 28 bp, synthetic construct
  source 1..28: mol_type = other DNA
tgaggcaggagaatcacttgaacctggg

SEQ ID NO: 29386 - DNA, 28 bp, synthetic construct
  source 1..28: mol_type = other DNA
ggcaggagaatcacttgaacctgggagg

SEQ ID NO: 29387 - DNA, 28 bp, synthetic construct
  source 1..28: mol_type = other DNA
aggagaatcacttgaacctgggaggcgg

SEQ ID NO: 29388 - DNA, 28 bp, synthetic construct
  source 1..28: mol_type = other DNA
agaatcacttgaacctgggaggcggagg

SEQ ID NO: 29389 - DNA, 28 bp, synthetic construct
  source 1..28: mol_type = other DNA
tggcttactgaaacctccgcctcccagg

SEQ ID NO: 29390 - DNA, 28 bp, synthetic construct
  source 1..28: mol_type = other DNA
aggctggaatgcagtggcgcgatcttgg

SEQ ID NO: 29391 - DNA, 28 bp, synthetic construct
  source 1..28: mol_type = other DNA
aagatcgcgccactgcattccagcctgg

SEQ ID NO: 29392 - DNA, 28 bp, synthetic construct
  source 1..28: mol_type = other DNA
agatcgcgccactgcattccagcctggg

SEQ ID NO: 29393 - DNA, 28 bp, synthetic construct
  source 1..28: mol_type = other DNA
cattgttgcccaggctggaatgcagtgg

SEQ ID NO: 29394 - DNA, 28 bp, synthetic construct
  source 1..28: mol_type = other DNA
gagtttcgctcattgttgcccaggctgg

SEQ ID NO: 29395 - DNA, 28 bp, synthetic construct
  source 1..28: mol_type = other DNA
gatggagtttcgctcattgttgcccagg

SEQ ID NO: 29396 - DNA, 28 bp, synthetic construct
  source 1..28: mol_type = other DNA
tttttttttttttttttttttgagatgg

SEQ ID NO: 29397 - DNA, 28 bp, synthetic construct
  source 1..28: mol_type = other DNA
aaaaaaaaaaaaaaaaaaaatgaccagg

SEQ ID NO: 29398 - DNA, 28 bp, synthetic construct
  source 1..28: mol_type = other DNA
ttcagtttgcaaagctgaaactgcctgg

SEQ ID NO: 29399 - DNA, 28 bp, synthetic construct
  source 1..28: mol_type = other DNA
cagctttgcaaactgaaaagagctgtgg

SEQ ID NO: 29400 - DNA, 28 bp, synthetic construct
  source 1..28: mol_type = other DNA
gcaaactgaaaagagctgtggagattgg

SEQ ID NO: 29401 - DNA, 28 bp, synthetic construct
  source 1..28: mol_type = other DNA
tgcgtacacttaaaaatagcgaagatgg

SEQ ID NO: 29402 - DNA, 28 bp, synthetic construct
  source 1..28: mol_type = other DNA
ttttaccacaattttttaaatgacaagg

SEQ ID NO: 29403 - DNA, 28 bp, synthetic construct
  source 1..28: mol_type = other DNA
atcttccttgtcatttaaaaaattgtgg

SEQ ID NO: 29404 - DNA, 28 bp, synthetic construct
  source 1..28: mol_type = other DNA
aaagctaaaaatagaattagtgaattgg

SEQ ID NO: 29405 - DNA, 28 bp, synthetic construct
  source 1..28: mol_type = other DNA
ctaaaaatagaattagtgaattggaagg

SEQ ID NO: 29406 - DNA, 28 bp, synthetic construct
  source 1..28: mol_type = other DNA
ggaagaaatgaaaaaattacctaaaagg

SEQ ID NO: 29407 - DNA, 28 bp, synthetic construct
  source 1..28: mol_type = other DNA
acctaaaaggcaatacagtaagacaagg

SEQ ID NO: 29408 - DNA, 28 bp, synthetic construct
  source 1..28: mol_type = other DNA
tccttgtcttactgtattgccttttagg

SEQ ID NO: 29409 - DNA, 28 bp, synthetic construct
  source 1..28: mol_type = other DNA
aaatataaagaaatgttaacctaaatgg

SEQ ID NO: 29410 - DNA, 28 bp, synthetic construct
  source 1..28: mol_type = other DNA
aacctaaatggagaatacaatgagaagg

SEQ ID NO: 29411 - DNA, 28 bp, synthetic construct
  source 1..28: mol_type = other DNA
gaccttctcattgtattctccatttagg

SEQ ID NO: 29412 - DNA, 28 bp, synthetic construct
  source 1..28: mol_type = other DNA
tgagaaggtccaaaatatgtctcatcgg

SEQ ID NO: 29413 - DNA, 28 bp, synthetic construct
  source 1..28: mol_type = other DNA
tctaggtctccgatgagacatattttgg

SEQ ID NO: 29414 - DNA, 28 bp, synthetic construct
  source 1..28: mol_type = other DNA
ggagacctagaagaaaagaatagaaagg

SEQ ID NO: 29415 - DNA, 28 bp, synthetic construct
  source 1..28: mol_type = other DNA
acctagaagaaaagaatagaaaggaagg

SEQ ID NO: 29416 - DNA, 28 bp, synthetic construct
  source 1..28: mol_type = other DNA
tccttcctttctattcttttcttctagg

SEQ ID NO: 29417 - DNA, 28 bp, synthetic construct
  source 1..28: mol_type = other DNA
tagaagaaaagaatagaaaggaaggagg

SEQ ID NO: 29418 - DNA, 28 bp, synthetic construct
  source 1..28: mol_type = other DNA
gaaaagaatagaaaggaaggaggaaagg

SEQ ID NO: 29419 - DNA, 28 bp, synthetic construct
  source 1..28: mol_type = other DNA
aaaagaatagaaaggaaggaggaaaggg

SEQ ID NO: 29420 - DNA, 28 bp, synthetic construct
  source 1..28: mol_type = other DNA
aaggaaggaggaaagggaatatttaagg

SEQ ID NO: 29421 - DNA, 28 bp, synthetic construct
  source 1..28: mol_type = other DNA
aggagatgataactgagatgtttccagg

SEQ ID NO: 29422 - DNA, 28 bp, synthetic construct
  source 1..28: mol_type = other DNA
gtggatttatgtcttttaacactcctgg

SEQ ID NO: 29423 - DNA, 28 bp, synthetic construct
  source 1..28: mol_type = other DNA
acataaatccacagatatactaatcagg

SEQ ID NO: 29424 - DNA, 28 bp, synthetic construct
  source 1..28: mol_type = other DNA
cataaatccacagatatactaatcaggg

SEQ ID NO: 29425 - DNA, 28 bp, synthetic construct
  source 1..28: mol_type = other DNA
tcatttaccctgattagtatatctgtgg

SEQ ID NO: 29426 - DNA, 28 bp, synthetic construct
  source 1..28: mol_type = other DNA
aatcagggtaaatgaaaagaaattcagg

SEQ ID NO: 29427 - DNA, 28 bp, synthetic construct
  source 1..28: mol_type = other DNA
agggtaaatgaaaagaaattcaggctgg

SEQ ID NO: 29428 - DNA, 28 bp, synthetic construct
  source 1..28: mol_type = other DNA
gggtaaatgaaaagaaattcaggctggg

SEQ ID NO: 29429 - DNA, 28 bp, synthetic construct
  source 1..28: mol_type = other DNA
aatgaaaagaaattcaggctgggcgcgg

SEQ ID NO: 29430 - DNA, 28 bp, synthetic construct
  source 1..28: mol_type = other DNA
gaaaagaaattcaggctgggcgcggtgg

SEQ ID NO: 29431 - DNA, 28 bp, synthetic construct
  source 1..28: mol_type = other DNA
gctcacaccttaaaccccagaactttgg

SEQ ID NO: 29432 - DNA, 28 bp, synthetic construct
  source 1..28: mol_type = other DNA
ctcacaccttaaaccccagaactttggg

SEQ ID NO: 29433 - DNA, 28 bp, synthetic construct
  source 1..28: mol_type = other DNA
acaccttaaaccccagaactttgggagg

SEQ ID NO: 29434 - DNA, 28 bp, synthetic construct
  source 1..28: mol_type = other DNA
cagcctcccaaagttctggggtttaagg

SEQ ID NO: 29435 - DNA, 28 bp, synthetic construct
  source 1..28: mol_type = other DNA
taaaccccagaactttgggaggctgagg

SEQ ID NO: 29436 - DNA, 28 bp, synthetic construct
  source 1..28: mol_type = other DNA
accccagaactttgggaggctgaggcgg

SEQ ID NO: 29437 - DNA, 28 bp, synthetic construct
  source 1..28: mol_type = other DNA
cccgcctcagcctcccaaagttctgggg

SEQ ID NO: 29438 - DNA, 28 bp, synthetic construct
  source 1..28: mol_type = other DNA
acccgcctcagcctcccaaagttctggg

SEQ ID NO: 29439 - DNA, 28 bp, synthetic construct
  source 1..28: mol_type = other DNA
cacccgcctcagcctcccaaagttctgg

SEQ ID NO: 29440 - DNA, 28 bp, synthetic construct
  source 1..28: mol_type = other DNA
cagaactttgggaggctgaggcgggtgg

SEQ ID NO: 29441 - DNA, 28 bp, synthetic construct
  source 1..28: mol_type = other DNA
gaggctgaggcgggtggatcacctgagg

SEQ ID NO: 29442 - DNA, 28 bp, synthetic construct
  source 1..28: mol_type = other DNA
tgaggcgggtggatcacctgaggtcagg

SEQ ID NO: 29443 - DNA, 28 bp, synthetic construct
  source 1..28: mol_type = other DNA
aggatggtcttgaactcctgacctcagg

SEQ ID NO: 29444 - DNA, 28 bp, synthetic construct
  source 1..28: mol_type = other DNA
gagttcaagaccatcctgaccaacatgg

SEQ ID NO: 29445 - DNA, 28 bp, synthetic construct
  source 1..28: mol_type = other DNA
tggggtttctccatgttggtcaggatgg

SEQ ID NO: 29446 - DNA, 28 bp, synthetic construct
  source 1..28: mol_type = other DNA
gatatggggtttctccatgttggtcagg

SEQ ID NO: 29447 - DNA, 28 bp, synthetic construct
  source 1..28: mol_type = other DNA
tagtagatatggggtttctccatgttgg

SEQ ID NO: 29448 - DNA, 28 bp, synthetic construct
  source 1..28: mol_type = other DNA
taagtttgtatttttagtagatatgggg

SEQ ID NO: 29449 - DNA, 28 bp, synthetic construct
  source 1..28: mol_type = other DNA
ctaagtttgtatttttagtagatatggg

SEQ ID NO: 29450 - DNA, 28 bp, synthetic construct
  source 1..28: mol_type = other DNA
gctaagtttgtatttttagtagatatgg

SEQ ID NO: 29451 - DNA, 28 bp, synthetic construct
  source 1..28: mol_type = other DNA
tatctactaaaaatacaaacttagccgg

SEQ ID NO: 29452 - DNA, 28 bp, synthetic construct
  source 1..28: mol_type = other DNA
atctactaaaaatacaaacttagccggg

SEQ ID NO: 29453 - DNA, 28 bp, synthetic construct
  source 1..28: mol_type = other DNA
ctaaaaatacaaacttagccgggcatgg

SEQ ID NO: 29454 - DNA, 28 bp, synthetic construct
  source 1..28: mol_type = other DNA
aaaatacaaacttagccgggcatggtgg

SEQ ID NO: 29455 - DNA, 28 bp, synthetic construct
  source 1..28: mol_type = other DNA
gattacaggtgcatgccaccatgcccgg

SEQ ID NO: 29456 - DNA, 28 bp, synthetic construct
  source 1..28: mol_type = other DNA
gcatgcacctgtaatcccagctactcgg

SEQ ID NO: 29457 - DNA, 28 bp, synthetic construct
  source 1..28: mol_type = other DNA
catgcacctgtaatcccagctactcggg

SEQ ID NO: 29458 - DNA, 28 bp, synthetic construct
  source 1..28: mol_type = other DNA
gcacctgtaatcccagctactcgggagg

SEQ ID NO: 29459 - DNA, 28 bp, synthetic construct
  source 1..28: mol_type = other DNA
cagcctcccgagtagctgggattacagg

SEQ ID NO: 29460 - DNA, 28 bp, synthetic construct
  source 1..28: mol_type = other DNA
gtaatcccagctactcgggaggctgagg

SEQ ID NO: 29461 - DNA, 28 bp, synthetic construct
  source 1..28: mol_type = other DNA
ttctgcctcagcctcccgagtagctggg

SEQ ID NO: 29462 - DNA, 28 bp, synthetic construct
  source 1..28: mol_type = other DNA
cttctgcctcagcctcccgagtagctgg

SEQ ID NO: 29463 - DNA, 28 bp, synthetic construct
  source 1..28: mol_type = other DNA
ctgaggcagaagaatcacttgaacccgg

SEQ ID NO: 29464 - DNA, 28 bp, synthetic construct
  source 1..28: mol_type = other DNA
tgaggcagaagaatcacttgaacccggg

SEQ ID NO: 29465 - DNA, 28 bp, synthetic construct
  source 1..28: mol_type = other DNA
ggcagaagaatcacttgaacccgggagg

SEQ ID NO: 29466 - DNA, 28 bp, synthetic construct
  source 1..28: mol_type = other DNA
agaagaatcacttgaacccgggaggcgg

SEQ ID NO: 29467 - DNA, 28 bp, synthetic construct
  source 1..28: mol_type = other DNA
agaatcacttgaacccgggaggcggagg

SEQ ID NO: 29468 - DNA, 28 bp, synthetic construct
  source 1..28: mol_type = other DNA
cggctcactgcaacctccgcctcccggg

SEQ ID NO: 29469 - DNA, 28 bp, synthetic construct
  source 1..28: mol_type = other DNA
tcggctcactgcaacctccgcctcccgg

SEQ ID NO: 29470 - DNA, 28 bp, synthetic construct
  source 1..28: mol_type = other DNA
aggctggagtgcagtggcacgatctcgg

SEQ ID NO: 29471 - DNA, 28 bp, synthetic construct
  source 1..28: mol_type = other DNA
gagatcgtgccactgcactccagcctgg

SEQ ID NO: 29472 - DNA, 28 bp, synthetic construct
  source 1..28: mol_type = other DNA
agatcgtgccactgcactccagcctggg

SEQ ID NO: 29473 - DNA, 28 bp, synthetic construct
  source 1..28: mol_type = other DNA
tcttgttgcccaggctggagtgcagtgg

SEQ ID NO: 29474 - DNA, 28 bp, synthetic construct
  source 1..28: mol_type = other DNA
ggagttttgttcttgttgcccaggctgg

SEQ ID NO: 29475 - DNA, 28 bp, synthetic construct
  source 1..28: mol_type = other DNA
agacggagttttgttcttgttgcccagg

SEQ ID NO: 29476 - DNA, 28 bp, synthetic construct
  source 1..28: mol_type = other DNA
cttttcttttcttttttttttgagacgg

SEQ ID NO: 29477 - DNA, 28 bp, synthetic construct
  source 1..28: mol_type = other DNA
aaagaaaagaaaagaaattcaatctagg

SEQ ID NO: 29478 - DNA, 28 bp, synthetic construct
  source 1..28: mol_type = other DNA
agaaaagagatgttaaattgcaacaagg

SEQ ID NO: 29479 - DNA, 28 bp, synthetic construct
  source 1..28: mol_type = other DNA
gtcatatgctggctttgtgttttctggg

SEQ ID NO: 29480 - DNA, 28 bp, synthetic construct
  source 1..28: mol_type = other DNA
ggtcatatgctggctttgtgttttctgg

SEQ ID NO: 29481 - DNA, 28 bp, synthetic construct
  source 1..28: mol_type = other DNA
tttctcactgggtctggtcatatgctgg

SEQ ID NO: 29482 - DNA, 28 bp, synthetic construct
  source 1..28: mol_type = other DNA
aatagaagggatttctcactgggtctgg

SEQ ID NO: 29483 - DNA, 28 bp, synthetic construct
  source 1..28: mol_type = other DNA
taagaaatagaagggatttctcactggg

SEQ ID NO: 29484 - DNA, 28 bp, synthetic construct
  source 1..28: mol_type = other DNA
gtaagaaatagaagggatttctcactgg

SEQ ID NO: 29485 - DNA, 28 bp, synthetic construct
  source 1..28: mol_type = other DNA
gggtaggtgatagtaagaaatagaaggg

SEQ ID NO: 29486 - DNA, 28 bp, synthetic construct
  source 1..28: mol_type = other DNA
ggggtaggtgatagtaagaaatagaagg

SEQ ID NO: 29487 - DNA, 28 bp, synthetic construct
  source 1..28: mol_type = other DNA
gggagaaaaggagtagaggaggggtagg

SEQ ID NO: 29488 - DNA, 28 bp, synthetic construct
  source 1..28: mol_type = other DNA
gctggggagaaaaggagtagaggagggg

SEQ ID NO: 29489 - DNA, 28 bp, synthetic construct
  source 1..28: mol_type = other DNA
tgctggggagaaaaggagtagaggaggg

SEQ ID NO: 29490 - DNA, 28 bp, synthetic construct
  source 1..28: mol_type = other DNA
atgctggggagaaaaggagtagaggagg

SEQ ID NO: 29491 - DNA, 28 bp, synthetic construct
  source 1..28: mol_type = other DNA
tgaatgctggggagaaaaggagtagagg

SEQ ID NO: 29492 - DNA, 28 bp, synthetic construct
  source 1..28: mol_type = other DNA
tcattgagtgaatgctggggagaaaagg

SEQ ID NO: 29493 - DNA, 28 bp, synthetic construct
  source 1..28: mol_type = other DNA
actctttctcattgagtgaatgctgggg

SEQ ID NO: 29494 - DNA, 28 bp, synthetic construct
  source 1..28: mol_type = other DNA
tactctttctcattgagtgaatgctggg

SEQ ID NO: 29495 - DNA, 28 bp, synthetic construct
  source 1..28: mol_type = other DNA
ctactctttctcattgagtgaatgctgg

SEQ ID NO: 29496 - DNA, 28 bp, synthetic construct
  source 1..28: mol_type = other DNA
cattcactcaatgagaaagagtagctgg

SEQ ID NO: 29497 - DNA, 28 bp, synthetic construct
  source 1..28: mol_type = other DNA
actcaatgagaaagagtagctggagcgg

SEQ ID NO: 29498 - DNA, 28 bp, synthetic construct
  source 1..28: mol_type = other DNA
ctcaatgagaaagagtagctggagcggg

SEQ ID NO: 29499 - DNA, 28 bp, synthetic construct
  source 1..28: mol_type = other DNA
aatgagaaagagtagctggagcgggtgg

SEQ ID NO: 29500 - DNA, 28 bp, synthetic construct
  source 1..28: mol_type = other DNA
atgagaaagagtagctggagcgggtggg

SEQ ID NO: 29501 - DNA, 28 bp, synthetic construct
  source 1..28: mol_type = other DNA
tgagaaagagtagctggagcgggtgggg

SEQ ID NO: 29502 - DNA, 28 bp, synthetic construct
  source 1..28: mol_type = other DNA
taaacctacctcctcccacataatctgg

SEQ ID NO: 29503 - DNA, 28 bp, synthetic construct
  source 1..28: mol_type = other DNA
ccatccagattatgtgggaggaggtagg

SEQ ID NO: 29504 - DNA, 28 bp, synthetic construct
  source 1..28: mol_type = other DNA
gcatccatccagattatgtgggaggagg

SEQ ID NO: 29505 - DNA, 28 bp, synthetic construct
  source 1..28: mol_type = other DNA
taggcatccatccagattatgtgggagg

SEQ ID NO: 29506 - DNA, 28 bp, synthetic construct
  source 1..28: mol_type = other DNA
ctgtaggcatccatccagattatgtggg

SEQ ID NO: 29507 - DNA, 28 bp, synthetic construct
  source 1..28: mol_type = other DNA
gctgtaggcatccatccagattatgtgg

SEQ ID NO: 29508 - DNA, 28 bp, synthetic construct
  source 1..28: mol_type = other DNA
tggatgcctacagccatgtcttcaatgg

SEQ ID NO: 29509 - DNA, 28 bp, synthetic construct
  source 1..28: mol_type = other DNA
ggatgcctacagccatgtcttcaatggg

SEQ ID NO: 29510 - DNA, 28 bp, synthetic construct
  source 1..28: mol_type = other DNA
ccttgcccattgaagacatggctgtagg

SEQ ID NO: 29511 - DNA, 28 bp, synthetic construct
  source 1..28: mol_type = other DNA
agactttccttgcccattgaagacatgg

SEQ ID NO: 29512 - DNA, 28 bp, synthetic construct
  source 1..28: mol_type = other DNA
tatctgaattgctactaaattaagatgg

SEQ ID NO: 29513 - DNA, 28 bp, synthetic construct
  source 1..28: mol_type = other DNA
tcaacttaacacaactgtccaatgtagg

SEQ ID NO: 29514 - DNA, 28 bp, synthetic construct
  source 1..28: mol_type = other DNA
cacatgtctctctttcttcctacattgg

SEQ ID NO: 29515 - DNA, 28 bp, synthetic construct
  source 1..28: mol_type = other DNA
tttatcacaagctttttgttgaggaagg

SEQ ID NO: 29516 - DNA, 28 bp, synthetic construct
  source 1..28: mol_type = other DNA
ggaatttatcacaagctttttgttgagg

SEQ ID NO: 29517 - DNA, 28 bp, synthetic construct
  source 1..28: mol_type = other DNA
ctgcaacttgcaatgcataggtaacagg

SEQ ID NO: 29518 - DNA, 28 bp, synthetic construct
  source 1..28: mol_type = other DNA
gtttcttctgcaacttgcaatgcatagg

SEQ ID NO: 29519 - DNA, 28 bp, synthetic construct
  source 1..28: mol_type = other DNA
gaaagcaaatggtgagagatagacttgg

SEQ ID NO: 29520 - DNA, 28 bp, synthetic construct
  source 1..28: mol_type = other DNA
tctatctctcaccatttgctttcccagg

SEQ ID NO: 29521 - DNA, 28 bp, synthetic construct
  source 1..28: mol_type = other DNA
ctatctctcaccatttgctttcccaggg

SEQ ID NO: 29522 - DNA, 28 bp, synthetic construct
  source 1..28: mol_type = other DNA
tggtttttgaccctgggaaagcaaatgg

SEQ ID NO: 29523 - DNA, 28 bp, synthetic construct
  source 1..28: mol_type = other DNA
caagatgattgtggtttttgaccctggg

SEQ ID NO: 29524 - DNA, 28 bp, synthetic construct
  source 1..28: mol_type = other DNA
tcaagatgattgtggtttttgaccctgg

SEQ ID NO: 29525 - DNA, 28 bp, synthetic construct
  source 1..28: mol_type = other DNA
aaaaccacaatcatcttgataaacaagg

SEQ ID NO: 29526 - DNA, 28 bp, synthetic construct
  source 1..28: mol_type = other DNA
taggccttgtttatcaagatgattgtgg

SEQ ID NO: 29527 - DNA, 28 bp, synthetic construct
  source 1..28: mol_type = other DNA
tgacgatgtatttttgtatttgcatagg

SEQ ID NO: 29528 - DNA, 28 bp, synthetic construct
  source 1..28: mol_type = other DNA
ttagaaatgggatggaggtgagtgcagg

SEQ ID NO: 29529 - DNA, 28 bp, synthetic construct
  source 1..28: mol_type = other DNA
acgttgcatattagaaatgggatggagg

SEQ ID NO: 29530 - DNA, 28 bp, synthetic construct
  source 1..28: mol_type = other DNA
aatacgttgcatattagaaatgggatgg

SEQ ID NO: 29531 - DNA, 28 bp, synthetic construct
  source 1..28: mol_type = other DNA
agttaatacgttgcatattagaaatggg

SEQ ID NO: 29532 - DNA, 28 bp, synthetic construct
  source 1..28: mol_type = other DNA
cagttaatacgttgcatattagaaatgg

SEQ ID NO: 29533 - DNA, 28 bp, synthetic construct
  source 1..28: mol_type = other DNA
agcgtagatgcttttcacaatgagttgg

SEQ ID NO: 29534 - DNA, 28 bp, synthetic construct
  source 1..28: mol_type = other DNA
tccatatacatcagctagccagaaaagg

SEQ ID NO: 29535 - DNA, 28 bp, synthetic construct
  source 1..28: mol_type = other DNA
ccatatacatcagctagccagaaaaggg

SEQ ID NO: 29536 - DNA, 28 bp, synthetic construct
  source 1..28: mol_type = other DNA
catatacatcagctagccagaaaagggg

SEQ ID NO: 29537 - DNA, 28 bp, synthetic construct
  source 1..28: mol_type = other DNA
atacatcagctagccagaaaaggggagg

SEQ ID NO: 29538 - DNA, 28 bp, synthetic construct
  source 1..28: mol_type = other DNA
ttattcattatctcctccccttttctgg

SEQ ID NO: 29539 - DNA, 28 bp, synthetic construct
  source 1..28: mol_type = other DNA
gggaggagataatgaataatacccaagg

SEQ ID NO: 29540 - DNA, 28 bp, synthetic construct
  source 1..28: mol_type = other DNA
ggaggagataatgaataatacccaaggg

SEQ ID NO: 29541 - DNA, 28 bp, synthetic construct
  source 1..28: mol_type = other DNA
gagataatgaataatacccaagggaagg

SEQ ID NO: 29542 - DNA, 28 bp, synthetic construct
  source 1..28: mol_type = other DNA
ctgaaaaagggattttccttcccttggg

SEQ ID NO: 29543 - DNA, 28 bp, synthetic construct
  source 1..28: mol_type = other DNA
gctgaaaaagggattttccttcccttgg

SEQ ID NO: 29544 - DNA, 28 bp, synthetic construct
  source 1..28: mol_type = other DNA
agggaaggaaaatccctttttcagctgg

SEQ ID NO: 29545 - DNA, 28 bp, synthetic construct
  source 1..28: mol_type = other DNA
ggcatgacttaaaccagctgaaaaaggg

SEQ ID NO: 29546 - DNA, 28 bp, synthetic construct
  source 1..28: mol_type = other DNA
cggcatgacttaaaccagctgaaaaagg

SEQ ID NO: 29547 - DNA, 28 bp, synthetic construct
  source 1..28: mol_type = other DNA
atgcatagtgctgtgtgcacattatcgg

SEQ ID NO: 29548 - DNA, 28 bp, synthetic construct
  source 1..28: mol_type = other DNA
tctatgaactaattgaaaagctttatgg

SEQ ID NO: 29549 - DNA, 28 bp, synthetic construct
  source 1..28: mol_type = other DNA
tgaattatattttctgggagttagaagg

SEQ ID NO: 29550 - DNA, 28 bp, synthetic construct
  source 1..28: mol_type = other DNA
aaaatgtgcgtgaattatattttctggg

SEQ ID NO: 29551 - DNA, 28 bp, synthetic construct
  source 1..28: mol_type = other DNA
taaaatgtgcgtgaattatattttctgg

SEQ ID NO: 29552 - DNA, 28 bp, synthetic construct
  source 1..28: mol_type = other DNA
ggataatagctagcaggatgctgtgtgg

SEQ ID NO: 29553 - DNA, 28 bp, synthetic construct
  source 1..28: mol_type = other DNA
ttgtaaatgatggataatagctagcagg

SEQ ID NO: 29554 - DNA, 28 bp, synthetic construct
  source 1..28: mol_type = other DNA
atagacaaataacacttgtaaatgatgg

SEQ ID NO: 29555 - DNA, 28 bp, synthetic construct
  source 1..28: mol_type = other DNA
aatgacactaaagttttgaaaaacgagg

SEQ ID NO: 29556 - DNA, 28 bp, synthetic construct
  source 1..28: mol_type = other DNA
aaaacgaggctgctctgccttcttctgg

SEQ ID NO: 29557 - DNA, 28 bp, synthetic construct
  source 1..28: mol_type = other DNA
catttgttaaaacacagccagaagaagg

SEQ ID NO: 29558 - DNA, 28 bp, synthetic construct
  source 1..28: mol_type = other DNA
cttcttctggctgtgttttaacaaatgg

SEQ ID NO: 29559 - DNA, 28 bp, synthetic construct
  source 1..28: mol_type = other DNA
ttttaacaaatggtatcaatgcaaaagg

SEQ ID NO: 29560 - DNA, 28 bp, synthetic construct
  source 1..28: mol_type = other DNA
caaaagagcaataaatttttttaaaagg

SEQ ID NO: 29561 - DNA, 28 bp, synthetic construct
  source 1..28: mol_type = other DNA
ccttcagacatttggctatctagacagg

SEQ ID NO: 29562 - DNA, 28 bp, synthetic construct
  source 1..28: mol_type = other DNA
cattgtgtatcagccttcagacatttgg

SEQ ID NO: 29563 - DNA, 28 bp, synthetic construct
  source 1..28: mol_type = other DNA
ctgaaggctgatacacaatgaaataagg

SEQ ID NO: 29564 - DNA, 28 bp, synthetic construct
  source 1..28: mol_type = other DNA
tgaaggctgatacacaatgaaataaggg

SEQ ID NO: 29565 - DNA, 28 bp, synthetic construct
  source 1..28: mol_type = other DNA
tttcttttagagataatgatctttaggg

SEQ ID NO: 29566 - DNA, 28 bp, synthetic construct
  source 1..28: mol_type = other DNA
ttttcttttagagataatgatctttagg

SEQ ID NO: 29567 - DNA, 28 bp, synthetic construct
  source 1..28: mol_type = other DNA
ctacattttatgcatctctttttgctgg

SEQ ID NO: 29568 - DNA, 28 bp, synthetic construct
  source 1..28: mol_type = other DNA
aagcaaaacagtttatgttgtaaaaggg

SEQ ID NO: 29569 - DNA, 28 bp, synthetic construct
  source 1..28: mol_type = other DNA
taagcaaaacagtttatgttgtaaaagg

SEQ ID NO: 29570 - DNA, 28 bp, synthetic construct
  source 1..28: mol_type = other DNA
atgttttagtcatggttgtcagttgtgg

SEQ ID NO: 29571 - DNA, 28 bp, synthetic construct
  source 1..28: mol_type = other DNA
caaccatgactaaaacatgaattctagg

SEQ ID NO: 29572 - DNA, 28 bp, synthetic construct
  source 1..28: mol_type = other DNA
aatcctagaattcatgttttagtcatgg

SEQ ID NO: 29573 - DNA, 28 bp, synthetic construct
  source 1..28: mol_type = other DNA
tctaggattaacattaaaataattttgg

SEQ ID NO: 29574 - DNA, 28 bp, synthetic construct
  source 1..28: mol_type = other DNA
ctaggattaacattaaaataattttggg

SEQ ID NO: 29575 - DNA, 28 bp, synthetic construct
  source 1..28: mol_type = other DNA
taacattaaaataattttgggacagagg

SEQ ID NO: 29576 - DNA, 28 bp, synthetic construct
  source 1..28: mol_type = other DNA
aacattaaaataattttgggacagaggg

SEQ ID NO: 29577 - DNA, 28 bp, synthetic construct
  source 1..28: mol_type = other DNA
cagaacccttccatttttcttttgctgg

SEQ ID NO: 29578 - DNA, 28 bp, synthetic construct
  source 1..28: mol_type = other DNA
agataccagcaaaagaaaaatggaaggg

SEQ ID NO: 29579 - DNA, 28 bp, synthetic construct
  source 1..28: mol_type = other DNA
aagataccagcaaaagaaaaatggaagg

SEQ ID NO: 29580 - DNA, 28 bp, synthetic construct
  source 1..28: mol_type = other DNA
ggataagataccagcaaaagaaaaatgg

SEQ ID NO: 29581 - DNA, 28 bp, synthetic construct
  source 1..28: mol_type = other DNA
agtggaagaacaaaactagtgtaggtgg

SEQ ID NO: 29582 - DNA, 28 bp, synthetic construct
  source 1..28: mol_type = other DNA
ttgagtggaagaacaaaactagtgtagg

SEQ ID NO: 29583 - DNA, 28 bp, synthetic construct
  source 1..28: mol_type = other DNA
tatcttttgagaatagatttttgagtgg

SEQ ID NO: 29584 - DNA, 28 bp, synthetic construct
  source 1..28: mol_type = other DNA
ctaaatgcattatcttcaagtagtttgg

SEQ ID NO: 29585 - DNA, 28 bp, synthetic construct
  source 1..28: mol_type = other DNA
aagttaattttatatcttcttttcttgg

SEQ ID NO: 29586 - DNA, 28 bp, synthetic construct
  source 1..28: mol_type = other DNA
aatgtcagctgtctgctggcatgattgg

SEQ ID NO: 29587 - DNA, 28 bp, synthetic construct
  source 1..28: mol_type = other DNA
agctgtaataatgtcagctgtctgctgg

SEQ ID NO: 29588 - DNA, 28 bp, synthetic construct
  source 1..28: mol_type = other DNA
agttaagcaagaaaagaaatgaagaagg

SEQ ID NO: 29589 - DNA, 28 bp, synthetic construct
  source 1..28: mol_type = other DNA
agaaatgaagaaggcaattatatagtgg

SEQ ID NO: 29590 - DNA, 28 bp, synthetic construct
  source 1..28: mol_type = other DNA
aacattgactacaaatgtgcttcttggg

SEQ ID NO: 29591 - DNA, 28 bp, synthetic construct
  source 1..28: mol_type = other DNA
caacattgactacaaatgtgcttcttgg

SEQ ID NO: 29592 - DNA, 28 bp, synthetic construct
  source 1..28: mol_type = other DNA
atgttgctaaacagtagttcactcgtgg

SEQ ID NO: 29593 - DNA, 28 bp, synthetic construct
  source 1..28: mol_type = other DNA
gccccctccccctgccagatatttttgg

SEQ ID NO: 29594 - DNA, 28 bp, synthetic construct
  source 1..28: mol_type = other DNA
ccccctccccctgccagatatttttggg

SEQ ID NO: 29595 - DNA, 28 bp, synthetic construct
  source 1..28: mol_type = other DNA
cccctccccctgccagatatttttgggg

SEQ ID NO: 29596 - DNA, 28 bp, synthetic construct
  source 1..28: mol_type = other DNA
accccaaaaatatctggcagggggaggg

SEQ ID NO: 29597 - DNA, 28 bp, synthetic construct
  source 1..28: mol_type = other DNA
aaccccaaaaatatctggcagggggagg

SEQ ID NO: 29598 - DNA, 28 bp, synthetic construct
  source 1..28: mol_type = other DNA
cacaaccccaaaaatatctggcaggggg

SEQ ID NO: 29599 - DNA, 28 bp, synthetic construct
  source 1..28: mol_type = other DNA
tcacaaccccaaaaatatctggcagggg

SEQ ID NO: 29600 - DNA, 28 bp, synthetic construct
  source 1..28: mol_type = other DNA
ctcacaaccccaaaaatatctggcaggg

SEQ ID NO: 29601 - DNA, 28 bp, synthetic construct
  source 1..28: mol_type = other DNA
actcacaaccccaaaaatatctggcagg

SEQ ID NO: 29602 - DNA, 28 bp, synthetic construct
  source 1..28: mol_type = other DNA
caaaactcacaaccccaaaaatatctgg

SEQ ID NO: 29603 - DNA, 28 bp, synthetic construct
  source 1..28: mol_type = other DNA
gatatttttggggttgtgagttttgagg

SEQ ID NO: 29604 - DNA, 28 bp, synthetic construct
  source 1..28: mol_type = other DNA
atatttttggggttgtgagttttgaggg

SEQ ID NO: 29605 - DNA, 28 bp, synthetic construct
  source 1..28: mol_type = other DNA
tatttttggggttgtgagttttgagggg

SEQ ID NO: 29606 - DNA, 28 bp, synthetic construct
  source 1..28: mol_type = other DNA
aaattacagttcattgatttcttgctgg

SEQ ID NO: 29607 - DNA, 28 bp, synthetic construct
  source 1..28: mol_type = other DNA
ttttaactcattttactgtttactttgg

SEQ ID NO: 29608 - DNA, 28 bp, synthetic construct
  source 1..28: mol_type = other DNA
tactattttatagcttaatgtcatatgg

SEQ ID NO: 29609 - DNA, 28 bp, synthetic construct
  source 1..28: mol_type = other DNA
agctataaaatagtactgaatcaaacgg

SEQ ID NO: 29610 - DNA, 28 bp, synthetic construct
  source 1..28: mol_type = other DNA
gaatcaaacggagagtagaatactttgg

SEQ ID NO: 29611 - DNA, 28 bp, synthetic construct
  source 1..28: mol_type = other DNA
tcaaacggagagtagaatactttggagg

SEQ ID NO: 29612 - DNA, 28 bp, synthetic construct
  source 1..28: mol_type = other DNA
acggagagtagaatactttggaggaagg

SEQ ID NO: 29613 - DNA, 28 bp, synthetic construct
  source 1..28: mol_type = other DNA
cggagagtagaatactttggaggaaggg

SEQ ID NO: 29614 - DNA, 28 bp, synthetic construct
  source 1..28: mol_type = other DNA
ggagagtagaatactttggaggaagggg

SEQ ID NO: 29615 - DNA, 28 bp, synthetic construct
  source 1..28: mol_type = other DNA
gagtagaatactttggaggaaggggtgg

SEQ ID NO: 29616 - DNA, 28 bp, synthetic construct
  source 1..28: mol_type = other DNA
tggtatctgaatatctatagacatttgg

SEQ ID NO: 29617 - DNA, 28 bp, synthetic construct
  source 1..28: mol_type = other DNA
acgagccagtgacgaatgaagacacagg

SEQ ID NO: 29618 - DNA, 28 bp, synthetic construct
  source 1..28: mol_type = other DNA
cgagccagtgacgaatgaagacacaggg

SEQ ID NO: 29619 - DNA, 28 bp, synthetic construct
  source 1..28: mol_type = other DNA
agttccctgtgtcttcattcgtcactgg

SEQ ID NO: 29620 - DNA, 28 bp, synthetic construct
  source 1..28: mol_type = other DNA
aagacacagggaactgagctgagcttgg

SEQ ID NO: 29621 - DNA, 28 bp, synthetic construct
  source 1..28: mol_type = other DNA
aagtggcagggaacagaagagggtgtgg

SEQ ID NO: 29622 - DNA, 28 bp, synthetic construct
  source 1..28: mol_type = other DNA
tattcaagtggcagggaacagaagaggg

SEQ ID NO: 29623 - DNA, 28 bp, synthetic construct
  source 1..28: mol_type = other DNA
ttattcaagtggcagggaacagaagagg

SEQ ID NO: 29624 - DNA, 28 bp, synthetic construct
  source 1..28: mol_type = other DNA
cattttggctcttattcaagtggcaggg

SEQ ID NO: 29625 - DNA, 28 bp, synthetic construct
  source 1..28: mol_type = other DNA
gcattttggctcttattcaagtggcagg

SEQ ID NO: 29626 - DNA, 28 bp, synthetic construct
  source 1..28: mol_type = other DNA
agtggcattttggctcttattcaagtgg

SEQ ID NO: 29627 - DNA, 28 bp, synthetic construct
  source 1..28: mol_type = other DNA
gaaaataagattagaagtggcattttgg

SEQ ID NO: 29628 - DNA, 28 bp, synthetic construct
  source 1..28: mol_type = other DNA
aagaaatggaaaataagattagaagtgg

SEQ ID NO: 29629 - DNA, 28 bp, synthetic construct
  source 1..28: mol_type = other DNA
gagttaataaaacacatttaagaaatgg

SEQ ID NO: 29630 - DNA, 28 bp, synthetic construct
  source 1..28: mol_type = other DNA
agaatatttagctttgcaataaaagagg

SEQ ID NO: 29631 - DNA, 28 bp, synthetic construct
  source 1..28: mol_type = other DNA
ttattgcaaagctaaatattctaattgg

SEQ ID NO: 29632 - DNA, 28 bp, synthetic construct
  source 1..28: mol_type = other DNA
gtgtttgtaatgctctgcagcagtgagg

SEQ ID NO: 29633 - DNA, 28 bp, synthetic construct
  source 1..28: mol_type = other DNA
gtaatgctctgcagcagtgaggttctgg

SEQ ID NO: 29634 - DNA, 28 bp, synthetic construct
  source 1..28: mol_type = other DNA
cagtgaggttctggcagacccagtgagg

SEQ ID NO: 29635 - DNA, 28 bp, synthetic construct
  source 1..28: mol_type = other DNA
gtgaagaaataaatgggacctcactggg

SEQ ID NO: 29636 - DNA, 28 bp, synthetic construct
  source 1..28: mol_type = other DNA
agtgaagaaataaatgggacctcactgg

SEQ ID NO: 29637 - DNA, 28 bp, synthetic construct
  source 1..28: mol_type = other DNA
cattattacaagtgaagaaataaatggg

SEQ ID NO: 29638 - DNA, 28 bp, synthetic construct
  source 1..28: mol_type = other DNA
ccatttatttcttcacttgtaataatgg

SEQ ID NO: 29639 - DNA, 28 bp, synthetic construct
  source 1..28: mol_type = other DNA
actactgtgttctgatgcactactcagg

SEQ ID NO: 29640 - DNA, 28 bp, synthetic construct
  source 1..28: mol_type = other DNA
tttcttcaaagcaatataactaagatgg

SEQ ID NO: 29641 - DNA, 28 bp, synthetic construct
  source 1..28: mol_type = other DNA
cagatatcctttctactcattcaaaagg

SEQ ID NO: 29642 - DNA, 28 bp, synthetic construct
  source 1..28: mol_type = other DNA
cggttctccttttgaatgagtagaaagg

SEQ ID NO: 29643 - DNA, 28 bp, synthetic construct
  source 1..28: mol_type = other DNA
accgaacaatgctgattattcctgaagg

SEQ ID NO: 29644 - DNA, 28 bp, synthetic construct
  source 1..28: mol_type = other DNA
tccttcaggaataatcagcattgttcgg

SEQ ID NO: 29645 - DNA, 28 bp, synthetic construct
  source 1..28: mol_type = other DNA
tgctttgaaaatcaaaaggtccttcagg

SEQ ID NO: 29646 - DNA, 28 bp, synthetic construct
  source 1..28: mol_type = other DNA
actagcaaatgctttgaaaatcaaaagg

SEQ ID NO: 29647 - DNA, 28 bp, synthetic construct
  source 1..28: mol_type = other DNA
aattaatccacgcagcccctccgcaagg

SEQ ID NO: 29648 - DNA, 28 bp, synthetic construct
  source 1..28: mol_type = other DNA
tagttttccttgcggaggggctgcgtgg

SEQ ID NO: 29649 - DNA, 28 bp, synthetic construct
  source 1..28: mol_type = other DNA
gcagcccctccgcaaggaaaactagagg

SEQ ID NO: 29650 - DNA, 28 bp, synthetic construct
  source 1..28: mol_type = other DNA
ttctcctctagttttccttgcggagggg

SEQ ID NO: 29651 - DNA, 28 bp, synthetic construct
  source 1..28: mol_type = other DNA
gttctcctctagttttccttgcggaggg

SEQ ID NO: 29652 - DNA, 28 bp, synthetic construct
  source 1..28: mol_type = other DNA
agttctcctctagttttccttgcggagg

SEQ ID NO: 29653 - DNA, 28 bp, synthetic construct
  source 1..28: mol_type = other DNA
cgcagttctcctctagttttccttgcgg

SEQ ID NO: 29654 - DNA, 28 bp, synthetic construct
  source 1..28: mol_type = other DNA
gtactaacattttagagacaacaacagg

SEQ ID NO: 29655 - DNA, 28 bp, synthetic construct
  source 1..28: mol_type = other DNA
ctaacattttagagacaacaacaggagg

SEQ ID NO: 29656 - DNA, 28 bp, synthetic construct
  source 1..28: mol_type = other DNA
taacattttagagacaacaacaggaggg

SEQ ID NO: 29657 - DNA, 28 bp, synthetic construct
  source 1..28: mol_type = other DNA
aacattttagagacaacaacaggagggg

SEQ ID NO: 29658 - DNA, 28 bp, synthetic construct
  source 1..28: mol_type = other DNA
acaacaacaggaggggacagatatttgg

SEQ ID NO: 29659 - DNA, 28 bp, synthetic construct
  source 1..28: mol_type = other DNA
ttgtagaagctctcagacttttgtcagg

SEQ ID NO: 29660 - DNA, 28 bp, synthetic construct
  source 1..28: mol_type = other DNA
atatgaatcaagtgacattttctgcagg

SEQ ID NO: 29661 - DNA, 28 bp, synthetic construct
  source 1..28: mol_type = other DNA
tcacttgattcatatcttcaactccagg

SEQ ID NO: 29662 - DNA, 28 bp, synthetic construct
  source 1..28: mol_type = other DNA
cacttgattcatatcttcaactccaggg

SEQ ID NO: 29663 - DNA, 28 bp, synthetic construct
  source 1..28: mol_type = other DNA
cttcaactccagggttatgccctgaagg

SEQ ID NO: 29664 - DNA, 28 bp, synthetic construct
  source 1..28: mol_type = other DNA
gtgcatttccttcagggcataaccctgg

SEQ ID NO: 29665 - DNA, 28 bp, synthetic construct
  source 1..28: mol_type = other DNA
catcatcatgagtgcatttccttcaggg

SEQ ID NO: 29666 - DNA, 28 bp, synthetic construct
  source 1..28: mol_type = other DNA
acatcatcatgagtgcatttccttcagg

SEQ ID NO: 29667 - DNA, 28 bp, synthetic construct
  source 1..28: mol_type = other DNA
tcatgatgatgtgaactgcaattcgtgg

SEQ ID NO: 29668 - DNA, 28 bp, synthetic construct
  source 1..28: mol_type = other DNA
aagggggaatgaattatgggtaagatgg

SEQ ID NO: 29669 - DNA, 28 bp, synthetic construct
  source 1..28: mol_type = other DNA
tgctaggtaagggggaatgaattatggg

SEQ ID NO: 29670 - DNA, 28 bp, synthetic construct
  source 1..28: mol_type = other DNA
gtgctaggtaagggggaatgaattatgg

SEQ ID NO: 29671 - DNA, 28 bp, synthetic construct
  source 1..28: mol_type = other DNA
agatcttaaagtgtgctaggtaaggggg

SEQ ID NO: 29672 - DNA, 28 bp, synthetic construct
  source 1..28: mol_type = other DNA
cagatcttaaagtgtgctaggtaagggg

SEQ ID NO: 29673 - DNA, 28 bp, synthetic construct
  source 1..28: mol_type = other DNA
acagatcttaaagtgtgctaggtaaggg

SEQ ID NO: 29674 - DNA, 28 bp, synthetic construct
  source 1..28: mol_type = other DNA
aacagatcttaaagtgtgctaggtaagg

SEQ ID NO: 29675 - DNA, 28 bp, synthetic construct
  source 1..28: mol_type = other DNA
gcatgaacagatcttaaagtgtgctagg

SEQ ID NO: 29676 - DNA, 28 bp, synthetic construct
  source 1..28: mol_type = other DNA
ctttttttttttttttttaactatgtgg

SEQ ID NO: 29677 - DNA, 28 bp, synthetic construct
  source 1..28: mol_type = other DNA
cacatagttaaaaaaaaaaaaaaaaagg

SEQ ID NO: 29678 - DNA, 28 bp, synthetic construct
  source 1..28: mol_type = other DNA
atagttaaaaaaaaaaaaaaaaaggtgg

SEQ ID NO: 29679 - DNA, 28 bp, synthetic construct
  source 1..28: mol_type = other DNA
tagttaaaaaaaaaaaaaaaaaggtggg

SEQ ID NO: 29680 - DNA, 28 bp, synthetic construct
  source 1..28: mol_type = other DNA
agttaaaaaaaaaaaaaaaaaggtgggg

SEQ ID NO: 29681 - DNA, 28 bp, synthetic construct
  source 1..28: mol_type = other DNA
gttaaaaaaaaaaaaaaaaaggtggggg

SEQ ID NO: 29682 - DNA, 28 bp, synthetic construct
  source 1..28: mol_type = other DNA
ttaaaaaaaaaaaaaaaaaggtgggggg

SEQ ID NO: 29683 - DNA, 28 bp, synthetic construct
  source 1..28: mol_type = other DNA
aaaaaaaaaaaaaaaaggtggggggagg

SEQ ID NO: 29684 - DNA, 28 bp, synthetic construct
  source 1..28: mol_type = other DNA
aaaaaaaaaaaaaaaggtggggggaggg

SEQ ID NO: 29685 - DNA, 28 bp, synthetic construct
  source 1..28: mol_type = other DNA
gataatcctaaacccctttcgtcccagg

SEQ ID NO: 29686 - DNA, 28 bp, synthetic construct
  source 1..28: mol_type = other DNA
ctaagtcctgggacgaaaggggtttagg

SEQ ID NO: 29687 - DNA, 28 bp, synthetic construct
  source 1..28: mol_type = other DNA
agctttctaagtcctgggacgaaagggg

SEQ ID NO: 29688 - DNA, 28 bp, synthetic construct
  source 1..28: mol_type = other DNA
aagctttctaagtcctgggacgaaaggg

SEQ ID NO: 29689 - DNA, 28 bp, synthetic construct
  source 1..28: mol_type = other DNA
taagctttctaagtcctgggacgaaagg

SEQ ID NO: 29690 - DNA, 28 bp, synthetic construct
  source 1..28: mol_type = other DNA
ggaaaaaataagctttctaagtcctggg

SEQ ID NO: 29691 - DNA, 28 bp, synthetic construct
  source 1..28: mol_type = other DNA
tggaaaaaataagctttctaagtcctgg

SEQ ID NO: 29692 - DNA, 28 bp, synthetic construct
  source 1..28: mol_type = other DNA
tttttccagtccaatatacagccaaagg

SEQ ID NO: 29693 - DNA, 28 bp, synthetic construct
  source 1..28: mol_type = other DNA
tccagtccaatatacagccaaaggaagg

SEQ ID NO: 29694 - DNA, 28 bp, synthetic construct
  source 1..28: mol_type = other DNA
tccttcctttggctgtatattggactgg

SEQ ID NO: 29695 - DNA, 28 bp, synthetic construct
  source 1..28: mol_type = other DNA
ccaatatacagccaaaggaaggagcagg

SEQ ID NO: 29696 - DNA, 28 bp, synthetic construct
  source 1..28: mol_type = other DNA
ttgtagattatcctgctccttcctttgg

SEQ ID NO: 29697 - DNA, 28 bp, synthetic construct
  source 1..28: mol_type = other DNA
aaaggaaggagcaggataatctacaagg

SEQ ID NO: 29698 - DNA, 28 bp, synthetic construct
  source 1..28: mol_type = other DNA
aaggaaggagcaggataatctacaaggg

SEQ ID NO: 29699 - DNA, 28 bp, synthetic construct
  source 1..28: mol_type = other DNA
tgttctcaggaaggaaacagataagagg

SEQ ID NO: 29700 - DNA, 28 bp, synthetic construct
  source 1..28: mol_type = other DNA
tatctgtttccttcctgagaacaaatgg

SEQ ID NO: 29701 - DNA, 28 bp, synthetic construct
  source 1..28: mol_type = other DNA
atgcttggtccatttgttctcaggaagg

SEQ ID NO: 29702 - DNA, 28 bp, synthetic construct
  source 1..28: mol_type = other DNA
ctgtatgcttggtccatttgttctcagg

SEQ ID NO: 29703 - DNA, 28 bp, synthetic construct
  source 1..28: mol_type = other DNA
atgtgtacactcacatctgtatgcttgg

SEQ ID NO: 29704 - DNA, 28 bp, synthetic construct
  source 1..28: mol_type = other DNA
atttacttcagatgcactttgagagggg

SEQ ID NO: 29705 - DNA, 28 bp, synthetic construct
  source 1..28: mol_type = other DNA
aatttacttcagatgcactttgagaggg

SEQ ID NO: 29706 - DNA, 28 bp, synthetic construct
  source 1..28: mol_type = other DNA
taatttacttcagatgcactttgagagg

SEQ ID NO: 29707 - DNA, 28 bp, synthetic construct
  source 1..28: mol_type = other DNA
cagggaacagactgatcactcagaaagg

SEQ ID NO: 29708 - DNA, 28 bp, synthetic construct
  source 1..28: mol_type = other DNA
ctgagtgatcagtctgttccctgaaagg

SEQ ID NO: 29709 - DNA, 28 bp, synthetic construct
  source 1..28: mol_type = other DNA
tgttccctgaaaggtcagaattttctgg

SEQ ID NO: 29710 - DNA, 28 bp, synthetic construct
  source 1..28: mol_type = other DNA
tttaccagaaaattctgacctttcaggg

SEQ ID NO: 29711 - DNA, 28 bp, synthetic construct
  source 1..28: mol_type = other DNA
atttaccagaaaattctgacctttcagg

SEQ ID NO: 29712 - DNA, 28 bp, synthetic construct
  source 1..28: mol_type = other DNA
tgtcgttgttgctgtttagacagggtgg

SEQ ID NO: 29713 - DNA, 28 bp, synthetic construct
  source 1..28: mol_type = other DNA
tgttgtcgttgttgctgtttagacaggg

SEQ ID NO: 29714 - DNA, 28 bp, synthetic construct
  source 1..28: mol_type = other DNA
ttgttgtcgttgttgctgtttagacagg

SEQ ID NO: 29715 - DNA, 28 bp, synthetic construct
  source 1..28: mol_type = other DNA
ctaaattccattgataagccaatagtgg

SEQ ID NO: 29716 - DNA, 28 bp, synthetic construct
  source 1..28: mol_type = other DNA
attaatgccactattggcttatcaatgg

SEQ ID NO: 29717 - DNA, 28 bp, synthetic construct
  source 1..28: mol_type = other DNA
aagccaatagtggcattaataataatgg

SEQ ID NO: 29718 - DNA, 28 bp, synthetic construct
  source 1..28: mol_type = other DNA
ttgccattattattaatgccactattgg

SEQ ID NO: 29719 - DNA, 28 bp, synthetic construct
  source 1..28: mol_type = other DNA
atttttctagatatcttaagactctcgg

SEQ ID NO: 29720 - DNA, 28 bp, synthetic construct
  source 1..28: mol_type = other DNA
tcatggagagggatgataaaaatatggg

SEQ ID NO: 29721 - DNA, 28 bp, synthetic construct
  source 1..28: mol_type = other DNA
ctcatggagagggatgataaaaatatgg

SEQ ID NO: 29722 - DNA, 28 bp, synthetic construct
  source 1..28: mol_type = other DNA
catatttttatcatccctctccatgagg

SEQ ID NO: 29723 - DNA, 28 bp, synthetic construct
  source 1..28: mol_type = other DNA
tttttatcatccctctccatgaggtagg

SEQ ID NO: 29724 - DNA, 28 bp, synthetic construct
  source 1..28: mol_type = other DNA
ttttatcatccctctccatgaggtaggg

SEQ ID NO: 29725 - DNA, 28 bp, synthetic construct
  source 1..28: mol_type = other DNA
tcatccctctccatgaggtagggcaagg

SEQ ID NO: 29726 - DNA, 28 bp, synthetic construct
  source 1..28: mol_type = other DNA
catccctctccatgaggtagggcaaggg

SEQ ID NO: 29727 - DNA, 28 bp, synthetic construct
  source 1..28: mol_type = other DNA
gtacccttgccctacctcatggagaggg

SEQ ID NO: 29728 - DNA, 28 bp, synthetic construct
  source 1..28: mol_type = other DNA
agtacccttgccctacctcatggagagg

SEQ ID NO: 29729 - DNA, 28 bp, synthetic construct
  source 1..28: mol_type = other DNA
taataagtacccttgccctacctcatgg

SEQ ID NO: 29730 - DNA, 28 bp, synthetic construct
  source 1..28: mol_type = other DNA
taggacatagttctcttgtgaaataggg

SEQ ID NO: 29731 - DNA, 28 bp, synthetic construct
  source 1..28: mol_type = other DNA
ctaggacatagttctcttgtgaaatagg

SEQ ID NO: 29732 - DNA, 28 bp, synthetic construct
  source 1..28: mol_type = other DNA
gcttagacaagtcttttaattttctagg

SEQ ID NO: 29733 - DNA, 28 bp, synthetic construct
  source 1..28: mol_type = other DNA
taaaagacttgtctaagctctaaactgg

SEQ ID NO: 29734 - DNA, 28 bp, synthetic construct
  source 1..28: mol_type = other DNA
ttgtctaagctctaaactggtaacaagg

SEQ ID NO: 29735 - DNA, 28 bp, synthetic construct
  source 1..28: mol_type = other DNA
tggtaacaaggcagagacatgaatttgg

SEQ ID NO: 29736 - DNA, 28 bp, synthetic construct
  source 1..28: mol_type = other DNA
ggtaacaaggcagagacatgaatttggg

SEQ ID NO: 29737 - DNA, 28 bp, synthetic construct
  source 1..28: mol_type = other DNA
tccaaactctctgctaactaaataatgg

SEQ ID NO: 29738 - DNA, 28 bp, synthetic construct
  source 1..28: mol_type = other DNA
gccattatttagttagcagagagtttgg

SEQ ID NO: 29739 - DNA, 28 bp, synthetic construct
  source 1..28: mol_type = other DNA
ttgtgttgacttttgtatgtcttctggg

SEQ ID NO: 29740 - DNA, 28 bp, synthetic construct
  source 1..28: mol_type = other DNA
tttgtgttgacttttgtatgtcttctgg

SEQ ID NO: 29741 - DNA, 28 bp, synthetic construct
  source 1..28: mol_type = other DNA
tattgtaggcagtgtaaataacagctgg

SEQ ID NO: 29742 - DNA, 28 bp, synthetic construct
  source 1..28: mol_type = other DNA
tttttctggaacaaacatttattgtagg

SEQ ID NO: 29743 - DNA, 28 bp, synthetic construct
  source 1..28: mol_type = other DNA
ctcatcttgtttgaactattttttctgg

SEQ ID NO: 29744 - DNA, 28 bp, synthetic construct
  source 1..28: mol_type = other DNA
agatgagaaatagtttaaacacaaaagg

SEQ ID NO: 29745 - DNA, 28 bp, synthetic construct
  source 1..28: mol_type = other DNA
aaatagtttaaacacaaaaggctgaagg

SEQ ID NO: 29746 - DNA, 28 bp, synthetic construct
  source 1..28: mol_type = other DNA
aatagtttaaacacaaaaggctgaaggg

SEQ ID NO: 29747 - DNA, 28 bp, synthetic construct
  source 1..28: mol_type = other DNA
cacaaaaggctgaagggttcaatatagg

SEQ ID NO: 29748 - DNA, 28 bp, synthetic construct
  source 1..28: mol_type = other DNA
aaaaatatgtttgcttttaatacagtgg

SEQ ID NO: 29749 - DNA, 28 bp, synthetic construct
  source 1..28: mol_type = other DNA
aatatgtttgcttttaatacagtggagg

SEQ ID NO: 29750 - DNA, 28 bp, synthetic construct
  source 1..28: mol_type = other DNA
ttttaatacagtggaggaactgttcagg

SEQ ID NO: 29751 - DNA, 28 bp, synthetic construct
  source 1..28: mol_type = other DNA
tcaggaacagtttgttcttctgtaaagg

SEQ ID NO: 29752 - DNA, 28 bp, synthetic construct
  source 1..28: mol_type = other DNA
gaacagtttgttcttctgtaaaggctgg

SEQ ID NO: 29753 - DNA, 28 bp, synthetic construct
  source 1..28: mol_type = other DNA
aaggctggccttgttgtactgccgaagg

SEQ ID NO: 29754 - DNA, 28 bp, synthetic construct
  source 1..28: mol_type = other DNA
tcttgcggccttcggcagtacaacaagg

SEQ ID NO: 29755 - DNA, 28 bp, synthetic construct
  source 1..28: mol_type = other DNA
acgtagcttgtgatcttgcggccttcgg

SEQ ID NO: 29756 - DNA, 28 bp, synthetic construct
  source 1..28: mol_type = other DNA
gaaggccgcaagatcacaagctacgtgg

SEQ ID NO: 29757 - DNA, 28 bp, synthetic construct
  source 1..28: mol_type = other DNA
caattccacgtagcttgtgatcttgcgg

SEQ ID NO: 29758 - DNA, 28 bp, synthetic construct
  source 1..28: mol_type = other DNA
gtggaattgagacgccagctcgcttcgg

SEQ ID NO: 29759 - DNA, 28 bp, synthetic construct
  source 1..28: mol_type = other DNA
agaagttggttgtgccgaagcgagctgg

SEQ ID NO: 29760 - DNA, 28 bp, synthetic construct
  source 1..28: mol_type = other DNA
gaacttagagcattaagagagaagttgg

SEQ ID NO: 29761 - DNA, 28 bp, synthetic construct
  source 1..28: mol_type = other DNA
ttcaggtcaaagctatgaagaagacagg

SEQ ID NO: 29762 - DNA, 28 bp, synthetic construct
  source 1..28: mol_type = other DNA
ttgtcaaaaagatcattcatggttcagg

SEQ ID NO: 29763 - DNA, 28 bp, synthetic construct
  source 1..28: mol_type = other DNA
ttttgtttgtcaaaaagatcattcatgg

SEQ ID NO: 29764 - DNA, 28 bp, synthetic construct
  source 1..28: mol_type = other DNA
caaaatttaaatgtgtgttataaacagg

SEQ ID NO: 29765 - DNA, 28 bp, synthetic construct
  source 1..28: mol_type = other DNA
aaaatttaaatgtgtgttataaacaggg

SEQ ID NO: 29766 - DNA, 28 bp, synthetic construct
  source 1..28: mol_type = other DNA
ggagcaagtgtcctaattttgatacagg

SEQ ID NO: 29767 - DNA, 28 bp, synthetic construct
  source 1..28: mol_type = other DNA
gagcaagtgtcctaattttgatacaggg

SEQ ID NO: 29768 - DNA, 28 bp, synthetic construct
  source 1..28: mol_type = other DNA
tttcttagcaccctgtatcaaaattagg

SEQ ID NO: 29769 - DNA, 28 bp, synthetic construct
  source 1..28: mol_type = other DNA
gggtgctaagaaatacagaaaacaaagg

SEQ ID NO: 29770 - DNA, 28 bp, synthetic construct
  source 1..28: mol_type = other DNA
aatacagaaaacaaaggaaattaactgg

SEQ ID NO: 29771 - DNA, 28 bp, synthetic construct
  source 1..28: mol_type = other DNA
atacagaaaacaaaggaaattaactggg

SEQ ID NO: 29772 - DNA, 28 bp, synthetic construct
  source 1..28: mol_type = other DNA
acaaaggaaattaactgggagatccagg

SEQ ID NO: 29773 - DNA, 28 bp, synthetic construct
  source 1..28: mol_type = other DNA
caaaggaaattaactgggagatccaggg

SEQ ID NO: 29774 - DNA, 28 bp, synthetic construct
  source 1..28: mol_type = other DNA
aggaaattaactgggagatccagggagg

SEQ ID NO: 29775 - DNA, 28 bp, synthetic construct
  source 1..28: mol_type = other DNA
gtggcagattgtttcttagcctccctgg

SEQ ID NO: 29776 - DNA, 28 bp, synthetic construct
  source 1..28: mol_type = other DNA
gggaggctaagaaacaatctgccactgg

SEQ ID NO: 29777 - DNA, 28 bp, synthetic construct
  source 1..28: mol_type = other DNA
ggaggctaagaaacaatctgccactggg

SEQ ID NO: 29778 - DNA, 28 bp, synthetic construct
  source 1..28: mol_type = other DNA
cagaagctatggctgtttctcccagtgg

SEQ ID NO: 29779 - DNA, 28 bp, synthetic construct
  source 1..28: mol_type = other DNA
aaacagccatagcttctgatgagctagg

SEQ ID NO: 29780 - DNA, 28 bp, synthetic construct
  source 1..28: mol_type = other DNA
aatcttcctagctcatcagaagctatgg

SEQ ID NO: 29781 - DNA, 28 bp, synthetic construct
  source 1..28: mol_type = other DNA
cttctgatgagctaggaagattttgtgg

SEQ ID NO: 29782 - DNA, 28 bp, synthetic construct
  source 1..28: mol_type = other DNA
tggttgatatcacagctgtttgttgagg

SEQ ID NO: 29783 - DNA, 28 bp, synthetic construct
  source 1..28: mol_type = other DNA
atatcacagctgtttgttgaggctgtgg

SEQ ID NO: 29784 - DNA, 28 bp, synthetic construct
  source 1..28: mol_type = other DNA
tcacagctgtttgttgaggctgtggtgg

SEQ ID NO: 29785 - DNA, 28 bp, synthetic construct
  source 1..28: mol_type = other DNA
cacagctgtttgttgaggctgtggtggg

SEQ ID NO: 29786 - DNA, 28 bp, synthetic construct
  source 1..28: mol_type = other DNA
gctgtggtgggatttctttttcaagagg

SEQ ID NO: 29787 - DNA, 28 bp, synthetic construct
  source 1..28: mol_type = other DNA
ctgtggtgggatttctttttcaagaggg

SEQ ID NO: 29788 - DNA, 28 bp, synthetic construct
  source 1..28: mol_type = other DNA
tgggatttctttttcaagagggtgaagg

SEQ ID NO: 29789 - DNA, 28 bp, synthetic construct
  source 1..28: mol_type = other DNA
gggatttctttttcaagagggtgaaggg

SEQ ID NO: 29790 - DNA, 28 bp, synthetic construct
  source 1..28: mol_type = other DNA
aagagggtgaagggagatttgaacttgg

SEQ ID NO: 29791 - DNA, 28 bp, synthetic construct
  source 1..28: mol_type = other DNA
gcgcctgacacaattatcctaaagtagg

SEQ ID NO: 29792 - DNA, 28 bp, synthetic construct
  source 1..28: mol_type = other DNA
tttcctactttaggataattgtgtcagg

SEQ ID NO: 29793 - DNA, 28 bp, synthetic construct
  source 1..28: mol_type = other DNA
tatcctaaagtaggaaagcctcagttgg

SEQ ID NO: 29794 - DNA, 28 bp, synthetic construct
  source 1..28: mol_type = other DNA
cttccaactgaggctttcctactttagg

SEQ ID NO: 29795 - DNA, 28 bp, synthetic construct
  source 1..28: mol_type = other DNA
aaagtaggaaagcctcagttggaagagg

SEQ ID NO: 29796 - DNA, 28 bp, synthetic construct
  source 1..28: mol_type = other DNA
aaagaaactcatcctcttccaactgagg

SEQ ID NO: 29797 - DNA, 28 bp, synthetic construct
  source 1..28: mol_type = other DNA
ggatgagtttctttaaatagcccaaagg

SEQ ID NO: 29798 - DNA, 28 bp, synthetic construct
  source 1..28: mol_type = other DNA
gcccaaaggctgtgatgcgtaaaaaagg

SEQ ID NO: 29799 - DNA, 28 bp, synthetic construct
  source 1..28: mol_type = other DNA
tccttttttacgcatcacagcctttggg

SEQ ID NO: 29800 - DNA, 28 bp, synthetic construct
  source 1..28: mol_type = other DNA
gtccttttttacgcatcacagcctttgg

SEQ ID NO: 29801 - DNA, 28 bp, synthetic construct
  source 1..28: mol_type = other DNA
gcgtaaaaaaggacttgacttattctgg

SEQ ID NO: 29802 - DNA, 28 bp, synthetic construct
  source 1..28: mol_type = other DNA
cttgacttattctggatagctccagagg

SEQ ID NO: 29803 - DNA, 28 bp, synthetic construct
  source 1..28: mol_type = other DNA
ttgacttattctggatagctccagaggg

SEQ ID NO: 29804 - DNA, 28 bp, synthetic construct
  source 1..28: mol_type = other DNA
agctccagagggcaaaactagcaagtgg

SEQ ID NO: 29805 - DNA, 28 bp, synthetic construct
  source 1..28: mol_type = other DNA
ctggccacttgctagttttgccctctgg

SEQ ID NO: 29806 - DNA, 28 bp, synthetic construct
  source 1..28: mol_type = other DNA
agggcaaaactagcaagtggccagcagg

SEQ ID NO: 29807 - DNA, 28 bp, synthetic construct
  source 1..28: mol_type = other DNA
ctactctgagtatgtgtgttcctgctgg

SEQ ID NO: 29808 - DNA, 28 bp, synthetic construct
  source 1..28: mol_type = other DNA
agtagagcagagcttgctaataattagg

SEQ ID NO: 29809 - DNA, 28 bp, synthetic construct
  source 1..28: mol_type = other DNA
aattaggactgcctcatccatagcaagg

SEQ ID NO: 29810 - DNA, 28 bp, synthetic construct
  source 1..28: mol_type = other DNA
ctctgagtgttccttgctatggatgagg

SEQ ID NO: 29811 - DNA, 28 bp, synthetic construct
  source 1..28: mol_type = other DNA
ctcatccatagcaaggaacactcagagg

SEQ ID NO: 29812 - DNA, 28 bp, synthetic construct
  source 1..28: mol_type = other DNA
atgagcctctgagtgttccttgctatgg

SEQ ID NO: 29813 - DNA, 28 bp, synthetic construct
  source 1..28: mol_type = other DNA
gccgccgtgggggtggggtgggtcgggg

SEQ ID NO: 29814 - DNA, 28 bp, synthetic construct
  source 1..28: mol_type = other DNA
ggccgccgtgggggtggggtgggtcggg

SEQ ID NO: 29815 - DNA, 28 bp, synthetic construct
  source 1..28: mol_type = other DNA
cggccgccgtgggggtggggtgggtcgg

SEQ ID NO: 29816 - DNA, 28 bp, synthetic construct
  source 1..28: mol_type = other DNA
cgacccaccccacccccacggcggccgg

SEQ ID NO: 29817 - DNA, 28 bp, synthetic construct
  source 1..28: mol_type = other DNA
cggccggccgccgtgggggtggggtggg

SEQ ID NO: 29818 - DNA, 28 bp, synthetic construct
  source 1..28: mol_type = other DNA
gcggccggccgccgtgggggtggggtgg

SEQ ID NO: 29819 - DNA, 28 bp, synthetic construct
  source 1..28: mol_type = other DNA
cgggcggccggccgccgtgggggtgggg

SEQ ID NO: 29820 - DNA, 28 bp, synthetic construct
  source 1..28: mol_type = other DNA
cccacccccacggcggccggccgcccgg

SEQ ID NO: 29821 - DNA, 28 bp, synthetic construct
  source 1..28: mol_type = other DNA
tccgggcggccggccgccgtgggggtgg

SEQ ID NO: 29822 - DNA, 28 bp, synthetic construct
  source 1..28: mol_type = other DNA
ggctccgggcggccggccgccgtggggg

SEQ ID NO: 29823 - DNA, 28 bp, synthetic construct
  source 1..28: mol_type = other DNA
gggctccgggcggccggccgccgtgggg

SEQ ID NO: 29824 - DNA, 28 bp, synthetic construct
  source 1..28: mol_type = other DNA
ggggctccgggcggccggccgccgtggg

SEQ ID NO: 29825 - DNA, 28 bp, synthetic construct
  source 1..28: mol_type = other DNA
gggggctccgggcggccggccgccgtgg

SEQ ID NO: 29826 - DNA, 28 bp, synthetic construct
  source 1..28: mol_type = other DNA
acggcggccggccgcccggagcccccgg

SEQ ID NO: 29827 - DNA, 28 bp, synthetic construct
  source 1..28: mol_type = other DNA
gccggccgcccggagcccccggcccagg

SEQ ID NO: 29828 - DNA, 28 bp, synthetic construct
  source 1..28: mol_type = other DNA
acctgggccgggggctccgggcggccgg

SEQ ID NO: 29829 - DNA, 28 bp, synthetic construct
  source 1..28: mol_type = other DNA
cctcacctgggccgggggctccgggcgg

SEQ ID NO: 29830 - DNA, 28 bp, synthetic construct
  source 1..28: mol_type = other DNA
cgtcctcacctgggccgggggctccggg

SEQ ID NO: 29831 - DNA, 28 bp, synthetic construct
  source 1..28: mol_type = other DNA
gcgtcctcacctgggccgggggctccgg

SEQ ID NO: 29832 - DNA, 28 bp, synthetic construct
  source 1..28: mol_type = other DNA
agcccccggcccaggtgaggacgcgcgg

SEQ ID NO: 29833 - DNA, 28 bp, synthetic construct
  source 1..28: mol_type = other DNA
gcccccggcccaggtgaggacgcgcggg

SEQ ID NO: 29834 - DNA, 28 bp, synthetic construct
  source 1..28: mol_type = other DNA
gcccgcgcgtcctcacctgggccggggg

SEQ ID NO: 29835 - DNA, 28 bp, synthetic construct
  source 1..28: mol_type = other DNA
ggcccgcgcgtcctcacctgggccgggg

SEQ ID NO: 29836 - DNA, 28 bp, synthetic construct
  source 1..28: mol_type = other DNA
cggcccgcgcgtcctcacctgggccggg

SEQ ID NO: 29837 - DNA, 28 bp, synthetic construct
  source 1..28: mol_type = other DNA
gcggcccgcgcgtcctcacctgggccgg

SEQ ID NO: 29838 - DNA, 28 bp, synthetic construct
  source 1..28: mol_type = other DNA
cgcggcggcccgcgcgtcctcacctggg

SEQ ID NO: 29839 - DNA, 28 bp, synthetic construct
  source 1..28: mol_type = other DNA
ccaggtgaggacgcgcgggccgccgcgg

SEQ ID NO: 29840 - DNA, 28 bp, synthetic construct
  source 1..28: mol_type = other DNA
cgggagcggcgaggggcggccgcggcgg

SEQ ID NO: 29841 - DNA, 28 bp, synthetic construct
  source 1..28: mol_type = other DNA
gggcgggagcggcgaggggcggccgcgg

SEQ ID NO: 29842 - DNA, 28 bp, synthetic construct
  source 1..28: mol_type = other DNA
tcgggcgggcgggagcggcgaggggcgg

SEQ ID NO: 29843 - DNA, 28 bp, synthetic construct
  source 1..28: mol_type = other DNA
gcttcgggcgggcgggagcggcgagggg

SEQ ID NO: 29844 - DNA, 28 bp, synthetic construct
  source 1..28: mol_type = other DNA
cgcttcgggcgggcgggagcggcgaggg

SEQ ID NO: 29845 - DNA, 28 bp, synthetic construct
  source 1..28: mol_type = other DNA
cctcgccgctcccgcccgcccgaagcgg

SEQ ID NO: 29846 - DNA, 28 bp, synthetic construct
  source 1..28: mol_type = other DNA
gccgctcccgcccgcccgaagcggccgg

SEQ ID NO: 29847 - DNA, 28 bp, synthetic construct
  source 1..28: mol_type = other DNA
gccggccgcttcgggcgggcgggagcgg

SEQ ID NO: 29848 - DNA, 28 bp, synthetic construct
  source 1..28: mol_type = other DNA
tcccgcccgcccgaagcggccggcacgg

SEQ ID NO: 29849 - DNA, 28 bp, synthetic construct
  source 1..28: mol_type = other DNA
cccgcccgcccgaagcggccggcacggg

SEQ ID NO: 29850 - DNA, 28 bp, synthetic construct
  source 1..28: mol_type = other DNA
ccgcccgcccgaagcggccggcacgggg

SEQ ID NO: 29851 - DNA, 28 bp, synthetic construct
  source 1..28: mol_type = other DNA
agtccccgtgccggccgcttcgggcggg

SEQ ID NO: 29852 - DNA, 28 bp, synthetic construct
  source 1..28: mol_type = other DNA
aagtccccgtgccggccgcttcgggcgg

SEQ ID NO: 29853 - DNA, 28 bp, synthetic construct
  source 1..28: mol_type = other DNA
ggtaagtccccgtgccggccgcttcggg

SEQ ID NO: 29854 - DNA, 28 bp, synthetic construct
  source 1..28: mol_type = other DNA
tggtaagtccccgtgccggccgcttcgg

SEQ ID NO: 29855 - DNA, 28 bp, synthetic construct
  source 1..28: mol_type = other DNA
gagtcactgtggtaagtccccgtgccgg

SEQ ID NO: 29856 - DNA, 28 bp, synthetic construct
  source 1..28: mol_type = other DNA
cacggggacttaccacagtgactcgagg

SEQ ID NO: 29857 - DNA, 28 bp, synthetic construct
  source 1..28: mol_type = other DNA
ccacagtgactcgaggtcccattcctgg

SEQ ID NO: 29858 - DNA, 28 bp, synthetic construct
  source 1..28: mol_type = other DNA
tgactcgaggtcccattcctggagcagg

SEQ ID NO: 29859 - DNA, 28 bp, synthetic construct
  source 1..28: mol_type = other DNA
gactcgaggtcccattcctggagcaggg

SEQ ID NO: 29860 - DNA, 28 bp, synthetic construct
  source 1..28: mol_type = other DNA
ttcgacttagccctgctccaggaatggg

SEQ ID NO: 29861 - DNA, 28 bp, synthetic construct
  source 1..28: mol_type = other DNA
cttcgacttagccctgctccaggaatgg

SEQ ID NO: 29862 - DNA, 28 bp, synthetic construct
  source 1..28: mol_type = other DNA
gacagcttcgacttagccctgctccagg

SEQ ID NO: 29863 - DNA, 28 bp, synthetic construct
  source 1..28: mol_type = other DNA
agcagggctaagtcgaagctgtccatgg

SEQ ID NO: 29864 - DNA, 28 bp, synthetic construct
  source 1..28: mol_type = other DNA
agggctaagtcgaagctgtccatggtgg

SEQ ID NO: 29865 - DNA, 28 bp, synthetic construct
  source 1..28: mol_type = other DNA
gggctaagtcgaagctgtccatggtggg

SEQ ID NO: 29866 - DNA, 28 bp, synthetic construct
  source 1..28: mol_type = other DNA
ctaagtcgaagctgtccatggtgggagg

SEQ ID NO: 29867 - DNA, 28 bp, synthetic construct
  source 1..28: mol_type = other DNA
gcggcgacgctgacacctcccaccatgg

SEQ ID NO: 29868 - DNA, 28 bp, synthetic construct
  source 1..28: mol_type = other DNA
gccgccgccgctaccgccgccgccgagg

SEQ ID NO: 29869 - DNA, 28 bp, synthetic construct
  source 1..28: mol_type = other DNA
gcctcggcggcggcggtagcggcggcgg

SEQ ID NO: 29870 - DNA, 28 bp, synthetic construct
  source 1..28: mol_type = other DNA
cgagcctcggcggcggcggtagcggcgg

SEQ ID NO: 29871 - DNA, 28 bp, synthetic construct
  source 1..28: mol_type = other DNA
cgccgctaccgccgccgccgaggctcgg

SEQ ID NO: 29872 - DNA, 28 bp, synthetic construct
  source 1..28: mol_type = other DNA
gccgctaccgccgccgccgaggctcggg

SEQ ID NO: 29873 - DNA, 28 bp, synthetic construct
  source 1..28: mol_type = other DNA
gcccgagcctcggcggcggcggtagcgg

SEQ ID NO: 29874 - DNA, 28 bp, synthetic construct
  source 1..28: mol_type = other DNA
cgggcggcccgagcctcggcggcggcgg

SEQ ID NO: 29875 - DNA, 28 bp, synthetic construct
  source 1..28: mol_type = other DNA
gcgcgggcggcccgagcctcggcggcgg

SEQ ID NO: 29876 - DNA, 28 bp, synthetic construct
  source 1..28: mol_type = other DNA
agcgcgcgggcggcccgagcctcggcgg

SEQ ID NO: 29877 - DNA, 28 bp, synthetic construct
  source 1..28: mol_type = other DNA
tgcagcgcgcgggcggcccgagcctcgg

SEQ ID NO: 29878 - DNA, 28 bp, synthetic construct
  source 1..28: mol_type = other DNA
cgggccgcccgcgcgctgcaacgaaagg

SEQ ID NO: 29879 - DNA, 28 bp, synthetic construct
  source 1..28: mol_type = other DNA
ggcgcctttcgttgcagcgcgcgggcgg

SEQ ID NO: 29880 - DNA, 28 bp, synthetic construct
  source 1..28: mol_type = other DNA
agcggcgcctttcgttgcagcgcgcggg

SEQ ID NO: 29881 - DNA, 28 bp, synthetic construct
  source 1..28: mol_type = other DNA
gagcggcgcctttcgttgcagcgcgcgg

SEQ ID NO: 29882 - DNA, 28 bp, synthetic construct
  source 1..28: mol_type = other DNA
gcgctgcaacgaaaggcgccgctcaagg

SEQ ID NO: 29883 - DNA, 28 bp, synthetic construct
  source 1..28: mol_type = other DNA
tggcgcggctgggatgcaccttgagcgg

SEQ ID NO: 29884 - DNA, 28 bp, synthetic construct
  source 1..28: mol_type = other DNA
aaggtgcatcccagccgcgccagagcgg

SEQ ID NO: 29885 - DNA, 28 bp, synthetic construct
  source 1..28: mol_type = other DNA
gggcggcggccgctctggcgcggctggg

SEQ ID NO: 29886 - DNA, 28 bp, synthetic construct
  source 1..28: mol_type = other DNA
cgggcggcggccgctctggcgcggctgg

SEQ ID NO: 29887 - DNA, 28 bp, synthetic construct
  source 1..28: mol_type = other DNA
tgggcgggcggcggccgctctggcgcgg

SEQ ID NO: 29888 - DNA, 28 bp, synthetic construct
  source 1..28: mol_type = other DNA
ggcggtgggcgggcggcggccgctctgg

SEQ ID NO: 29889 - DNA, 28 bp, synthetic construct
  source 1..28: mol_type = other DNA
ctgggggtgggcggtgggcgggcggcgg

SEQ ID NO: 29890 - DNA, 28 bp, synthetic construct
  source 1..28: mol_type = other DNA
cgccgcccgcccaccgcccacccccagg

SEQ ID NO: 29891 - DNA, 28 bp, synthetic construct
  source 1..28: mol_type = other DNA
gacctgggggtgggcggtgggcgggcgg

SEQ ID NO: 29892 - DNA, 28 bp, synthetic construct
  source 1..28: mol_type = other DNA
gcccgcccaccgcccacccccaggtcgg

SEQ ID NO: 29893 - DNA, 28 bp, synthetic construct
  source 1..28: mol_type = other DNA
cccgacctgggggtgggcggtgggcggg

SEQ ID NO: 29894 - DNA, 28 bp, synthetic construct
  source 1..28: mol_type = other DNA
ccgcccaccgcccacccccaggtcgggg

SEQ ID NO: 29895 - DNA, 28 bp, synthetic construct
  source 1..28: mol_type = other DNA
gagccccgacctgggggtgggcggtggg

SEQ ID NO: 29896 - DNA, 28 bp, synthetic construct
  source 1..28: mol_type = other DNA
ggagccccgacctgggggtgggcggtgg

SEQ ID NO: 29897 - DNA, 28 bp, synthetic construct
  source 1..28: mol_type = other DNA
tcgggagccccgacctgggggtgggcgg

SEQ ID NO: 29898 - DNA, 28 bp, synthetic construct
  source 1..28: mol_type = other DNA
gcgtcgggagccccgacctgggggtggg

SEQ ID NO: 29899 - DNA, 28 bp, synthetic construct
  source 1..28: mol_type = other DNA
ggcgtcgggagccccgacctgggggtgg

SEQ ID NO: 29900 - DNA, 28 bp, synthetic construct
  source 1..28: mol_type = other DNA
gggggcgtcgggagccccgacctggggg

SEQ ID NO: 29901 - DNA, 28 bp, synthetic construct
  source 1..28: mol_type = other DNA
ggggggcgtcgggagccccgacctgggg

SEQ ID NO: 29902 - DNA, 28 bp, synthetic construct
  source 1..28: mol_type = other DNA
cggggggcgtcgggagccccgacctggg

SEQ ID NO: 29903 - DNA, 28 bp, synthetic construct
  source 1..28: mol_type = other DNA
gcggggggcgtcgggagccccgacctgg

SEQ ID NO: 29904 - DNA, 28 bp, synthetic construct
  source 1..28: mol_type = other DNA
tcccgacgccccccgcccccgactccgg

SEQ ID NO: 29905 - DNA, 28 bp, synthetic construct
  source 1..28: mol_type = other DNA
cccgacgccccccgcccccgactccggg

SEQ ID NO: 29906 - DNA, 28 bp, synthetic construct
  source 1..28: mol_type = other DNA
gcccggagtcgggggcggggggcgtcgg

SEQ ID NO: 29907 - DNA, 28 bp, synthetic construct
  source 1..28: mol_type = other DNA
acgccccccgcccccgactccgggccgg

SEQ ID NO: 29908 - DNA, 28 bp, synthetic construct
  source 1..28: mol_type = other DNA
cggccggcccggagtcgggggcgggggg

SEQ ID NO: 29909 - DNA, 28 bp, synthetic construct
  source 1..28: mol_type = other DNA
ccggccggcccggagtcgggggcggggg

SEQ ID NO: 29910 - DNA, 28 bp, synthetic construct
  source 1..28: mol_type = other DNA
ccccgcccccgactccgggccggccggg

SEQ ID NO: 29911 - DNA, 28 bp, synthetic construct
  source 1..28: mol_type = other DNA
gcccggccggcccggagtcgggggcggg

SEQ ID NO: 29912 - DNA, 28 bp, synthetic construct
  source 1..28: mol_type = other DNA
agcccggccggcccggagtcgggggcgg

SEQ ID NO: 29913 - DNA, 28 bp, synthetic construct
  source 1..28: mol_type = other DNA
gcccccgactccgggccggccgggctgg

SEQ ID NO: 29914 - DNA, 28 bp, synthetic construct
  source 1..28: mol_type = other DNA
gccagcccggccggcccggagtcggggg

SEQ ID NO: 29915 - DNA, 28 bp, synthetic construct
  source 1..28: mol_type = other DNA
agccagcccggccggcccggagtcgggg

SEQ ID NO: 29916 - DNA, 28 bp, synthetic construct
  source 1..28: mol_type = other DNA
cagccagcccggccggcccggagtcggg

SEQ ID NO: 29917 - DNA, 28 bp, synthetic construct
  source 1..28: mol_type = other DNA
gcagccagcccggccggcccggagtcgg

SEQ ID NO: 29918 - DNA, 28 bp, synthetic construct
  source 1..28: mol_type = other DNA
tccgggccggccgggctggctgcagcgg

SEQ ID NO: 29919 - DNA, 28 bp, synthetic construct
  source 1..28: mol_type = other DNA
gccgctgcagccagcccggccggcccgg

SEQ ID NO: 29920 - DNA, 28 bp, synthetic construct
  source 1..28: mol_type = other DNA
ggccggccgggctggctgcagcggccgg

SEQ ID NO: 29921 - DNA, 28 bp, synthetic construct
  source 1..28: mol_type = other DNA
cgccggccgctgcagccagcccggccgg

SEQ ID NO: 29922 - DNA, 28 bp, synthetic construct
  source 1..28: mol_type = other DNA
agtgcgccggccgctgcagccagcccgg

SEQ ID NO: 29923 - DNA, 28 bp, synthetic construct
  source 1..28: mol_type = other DNA
gcggccggcgcactcacccgctccccgg

SEQ ID NO: 29924 - DNA, 28 bp, synthetic construct
  source 1..28: mol_type = other DNA
caagccggggagcgggtgagtgcgccgg

SEQ ID NO: 29925 - DNA, 28 bp, synthetic construct
  source 1..28: mol_type = other DNA
ctcacccgctccccggcttgcgcgcagg

SEQ ID NO: 29926 - DNA, 28 bp, synthetic construct
  source 1..28: mol_type = other DNA
tgtgcctgcgcgcaagccggggagcggg

SEQ ID NO: 29927 - DNA, 28 bp, synthetic construct
  source 1..28: mol_type = other DNA
gtgtgcctgcgcgcaagccggggagcgg

SEQ ID NO: 29928 - DNA, 28 bp, synthetic construct
  source 1..28: mol_type = other DNA
cttgagtgtgcctgcgcgcaagccgggg

SEQ ID NO: 29929 - DNA, 28 bp, synthetic construct
  source 1..28: mol_type = other DNA
tcttgagtgtgcctgcgcgcaagccggg

SEQ ID NO: 29930 - DNA, 28 bp, synthetic construct
  source 1..28: mol_type = other DNA
ctcttgagtgtgcctgcgcgcaagccgg

SEQ ID NO: 29931 - DNA, 28 bp, synthetic construct
  source 1..28: mol_type = other DNA
ccgggggcggggggcggcggcggcgcgg

SEQ ID NO: 29932 - DNA, 28 bp, synthetic construct
  source 1..28: mol_type = other DNA
cagggccgggggcggggggcggcggcgg

SEQ ID NO: 29933 - DNA, 28 bp, synthetic construct
  source 1..28: mol_type = other DNA
gcgcagggccgggggcggggggcggcgg

SEQ ID NO: 29934 - DNA, 28 bp, synthetic construct
  source 1..28: mol_type = other DNA
cgggcgcagggccgggggcggggggcgg

SEQ ID NO: 29935 - DNA, 28 bp, synthetic construct
  source 1..28: mol_type = other DNA
gggcgggcgcagggccgggggcgggggg

SEQ ID NO: 29936 - DNA, 28 bp, synthetic construct
  source 1..28: mol_type = other DNA
ggggcgggcgcagggccgggggcggggg

SEQ ID NO: 29937 - DNA, 28 bp, synthetic construct
  source 1..28: mol_type = other DNA
aggggcgggcgcagggccgggggcgggg

SEQ ID NO: 29938 - DNA, 28 bp, synthetic construct
  source 1..28: mol_type = other DNA
gaggggcgggcgcagggccgggggcggg

SEQ ID NO: 29939 - DNA, 28 bp, synthetic construct
  source 1..28: mol_type = other DNA
ggaggggcgggcgcagggccgggggcgg

SEQ ID NO: 29940 - DNA, 28 bp, synthetic construct
  source 1..28: mol_type = other DNA
ggaggaggggcgggcgcagggccggggg

SEQ ID NO: 29941 - DNA, 28 bp, synthetic construct
  source 1..28: mol_type = other DNA
gggaggaggggcgggcgcagggccgggg

SEQ ID NO: 29942 - DNA, 28 bp, synthetic construct
  source 1..28: mol_type = other DNA
ggggaggaggggcgggcgcagggccggg

SEQ ID NO: 29943 - DNA, 28 bp, synthetic construct
  source 1..28: mol_type = other DNA
aggggaggaggggcgggcgcagggccgg

SEQ ID NO: 29944 - DNA, 28 bp, synthetic construct
  source 1..28: mol_type = other DNA
agggaggggaggaggggcgggcgcaggg

SEQ ID NO: 29945 - DNA, 28 bp, synthetic construct
  source 1..28: mol_type = other DNA
gagggaggggaggaggggcgggcgcagg

SEQ ID NO: 29946 - DNA, 28 bp, synthetic construct
  source 1..28: mol_type = other DNA
cgcccgcccctcctcccctccctcgcgg

SEQ ID NO: 29947 - DNA, 28 bp, synthetic construct
  source 1..28: mol_type = other DNA
cgccgcgagggaggggaggaggggcggg

SEQ ID NO: 29948 - DNA, 28 bp, synthetic construct
  source 1..28: mol_type = other DNA
ccgcccctcctcccctccctcgcggcgg

SEQ ID NO: 29949 - DNA, 28 bp, synthetic construct
  source 1..28: mol_type = other DNA
gggccgccgcgagggaggggaggagggg

SEQ ID NO: 29950 - DNA, 28 bp, synthetic construct
  source 1..28: mol_type = other DNA
cgggccgccgcgagggaggggaggaggg

SEQ ID NO: 29951 - DNA, 28 bp, synthetic construct
  source 1..28: mol_type = other DNA
cctcctcccctccctcgcggcggcccgg

SEQ ID NO: 29952 - DNA, 28 bp, synthetic construct
  source 1..28: mol_type = other DNA
gggccgggccgccgcgagggaggggagg

SEQ ID NO: 29953 - DNA, 28 bp, synthetic construct
  source 1..28: mol_type = other DNA
agcgggccgggccgccgcgagggagggg

SEQ ID NO: 29954 - DNA, 28 bp, synthetic construct
  source 1..28: mol_type = other DNA
cagcgggccgggccgccgcgagggaggg

SEQ ID NO: 29955 - DNA, 28 bp, synthetic construct
  source 1..28: mol_type = other DNA
gcagcgggccgggccgccgcgagggagg

SEQ ID NO: 29956 - DNA, 28 bp, synthetic construct
  source 1..28: mol_type = other DNA
gcagcagcgggccgggccgccgcgaggg

SEQ ID NO: 29957 - DNA, 28 bp, synthetic construct
  source 1..28: mol_type = other DNA
tgcagcagcgggccgggccgccgcgagg

SEQ ID NO: 29958 - DNA, 28 bp, synthetic construct
  source 1..28: mol_type = other DNA
gcggcggcggctgcagcagcgggccggg

SEQ ID NO: 29959 - DNA, 28 bp, synthetic construct
  source 1..28: mol_type = other DNA
ggcggcggcggctgcagcagcgggccgg

SEQ ID NO: 29960 - DNA, 28 bp, synthetic construct
  source 1..28: mol_type = other DNA
cggcggcggcggcggctgcagcagcggg

SEQ ID NO: 29961 - DNA, 28 bp, synthetic construct
  source 1..28: mol_type = other DNA
gcggcggcggcggcggctgcagcagcgg

SEQ ID NO: 29962 - DNA, 28 bp, synthetic construct
  source 1..28: mol_type = other DNA
gccgccgccgccgccgccgccgccgcgg

SEQ ID NO: 29963 - DNA, 28 bp, synthetic construct
  source 1..28: mol_type = other DNA
accgcggcggcggcggcggcggcggcgg

SEQ ID NO: 29964 - DNA, 28 bp, synthetic construct
  source 1..28: mol_type = other DNA
agcaccgcggcggcggcggcggcggcgg

SEQ ID NO: 29965 - DNA, 28 bp, synthetic construct
  source 1..28: mol_type = other DNA
cagagcaccgcggcggcggcggcggcgg

SEQ ID NO: 29966 - DNA, 28 bp, synthetic construct
  source 1..28: mol_type = other DNA
gcgcagagcaccgcggcggcggcggcgg

SEQ ID NO: 29967 - DNA, 28 bp, synthetic construct
  source 1..28: mol_type = other DNA
cgggcgcagagcaccgcggcggcggcgg

SEQ ID NO: 29968 - DNA, 28 bp, synthetic construct
  source 1..28: mol_type = other DNA
gggcgggcgcagagcaccgcggcggcgg

SEQ ID NO: 29969 - DNA, 28 bp, synthetic construct
  source 1..28: mol_type = other DNA
ggcgggcgggcgcagagcaccgcggcgg

SEQ ID NO: 29970 - DNA, 28 bp, synthetic construct
  source 1..28: mol_type = other DNA
gcgggcgggcgggcgcagagcaccgcgg

SEQ ID NO: 29971 - DNA, 28 bp, synthetic construct
  source 1..28: mol_type = other DNA
cccgcccgcccgcctctttctcctccgg

SEQ ID NO: 29972 - DNA, 28 bp, synthetic construct
  source 1..28: mol_type = other DNA
ccgcccgcccgcctctttctcctccggg

SEQ ID NO: 29973 - DNA, 28 bp, synthetic construct
  source 1..28: mol_type = other DNA
cccgcccgcctctttctcctccgggagg

SEQ ID NO: 29974 - DNA, 28 bp, synthetic construct
  source 1..28: mol_type = other DNA
gcctcccggaggagaaagaggcgggcgg

SEQ ID NO: 29975 - DNA, 28 bp, synthetic construct
  source 1..28: mol_type = other DNA
cgcgcctcccggaggagaaagaggcggg

SEQ ID NO: 29976 - DNA, 28 bp, synthetic construct
  source 1..28: mol_type = other DNA
acgcgcctcccggaggagaaagaggcgg

SEQ ID NO: 29977 - DNA, 28 bp, synthetic construct
  source 1..28: mol_type = other DNA
cacacgcgcctcccggaggagaaagagg

SEQ ID NO: 29978 - DNA, 28 bp, synthetic construct
  source 1..28: mol_type = other DNA
ttctcctccgggaggcgcgtgtgcgcgg

SEQ ID NO: 29979 - DNA, 28 bp, synthetic construct
  source 1..28: mol_type = other DNA
tctcctccgggaggcgcgtgtgcgcggg

SEQ ID NO: 29980 - DNA, 28 bp, synthetic construct
  source 1..28: mol_type = other DNA
tcgcccgcgcacacgcgcctcccggagg

SEQ ID NO: 29981 - DNA, 28 bp, synthetic construct
  source 1..28: mol_type = other DNA
tccgggaggcgcgtgtgcgcgggcgagg

SEQ ID NO: 29982 - DNA, 28 bp, synthetic construct
  source 1..28: mol_type = other DNA
gcctcgcccgcgcacacgcgcctcccgg

SEQ ID NO: 29983 - DNA, 28 bp, synthetic construct
  source 1..28: mol_type = other DNA
aggcgcgtgtgcgcgggcgaggccgagg

SEQ ID NO: 29984 - DNA, 28 bp, synthetic construct
  source 1..28: mol_type = other DNA
cggggctcacggtgcgcgcgcgcctcgg

SEQ ID NO: 29985 - DNA, 28 bp, synthetic construct
  source 1..28: mol_type = other DNA
cggggcgggcgcggcgcggggctcacgg

SEQ ID NO: 29986 - DNA, 28 bp, synthetic construct
  source 1..28: mol_type = other DNA
gggcgcgcggggcgggcgcggcgcgggg

SEQ ID NO: 29987 - DNA, 28 bp, synthetic construct
  source 1..28: mol_type = other DNA
ggggcgcgcggggcgggcgcggcgcggg

SEQ ID NO: 29988 - DNA, 28 bp, synthetic construct
  source 1..28: mol_type = other DNA
aggggcgcgcggggcgggcgcggcgcgg

SEQ ID NO: 29989 - DNA, 28 bp, synthetic construct
  source 1..28: mol_type = other DNA
agtacaggggcgcgcggggcgggcgcgg

SEQ ID NO: 29990 - DNA, 28 bp, synthetic construct
  source 1..28: mol_type = other DNA
cggggagtacaggggcgcgcggggcggg

SEQ ID NO: 29991 - DNA, 28 bp, synthetic construct
  source 1..28: mol_type = other DNA
gcggggagtacaggggcgcgcggggcgg

SEQ ID NO: 29992 - DNA, 28 bp, synthetic construct
  source 1..28: mol_type = other DNA
ggcgcggggagtacaggggcgcgcgggg

SEQ ID NO: 29993 - DNA, 28 bp, synthetic construct
  source 1..28: mol_type = other DNA
cggcgcggggagtacaggggcgcgcggg

SEQ ID NO: 29994 - DNA, 28 bp, synthetic construct
  source 1..28: mol_type = other DNA
gcggcgcggggagtacaggggcgcgcgg

SEQ ID NO: 29995 - DNA, 28 bp, synthetic construct
  source 1..28: mol_type = other DNA
ccgaggagcggcgcggggagtacagggg

SEQ ID NO: 29996 - DNA, 28 bp, synthetic construct
  source 1..28: mol_type = other DNA
cccgaggagcggcgcggggagtacaggg

SEQ ID NO: 29997 - DNA, 28 bp, synthetic construct
  source 1..28: mol_type = other DNA
cctgtactccccgcgccgctcctcgggg

SEQ ID NO: 29998 - DNA, 28 bp, synthetic construct
  source 1..28: mol_type = other DNA
ccgcgggaccccgaggagcggcgcgggg

SEQ ID NO: 29999 - DNA, 28 bp, synthetic construct
  source 1..28: mol_type = other DNA
gccgcgggaccccgaggagcggcgcggg

SEQ ID NO: 30000 - DNA, 28 bp, synthetic construct
  source 1..28: mol_type = other DNA
cgccgcgggaccccgaggagcggcgcgg

SEQ ID NO: 30001 - DNA, 28 bp, synthetic construct
  source 1..28: mol_type = other DNA
gcgagcgccgcgggaccccgaggagcgg

SEQ ID NO: 30002 - DNA, 28 bp, synthetic construct
  source 1..28: mol_type = other DNA
ctcctcggggtcccgcggcgctcgcagg

SEQ ID NO: 30003 - DNA, 28 bp, synthetic construct
  source 1..28: mol_type = other DNA
ggcctgcgagcgccgcgggaccccgagg

SEQ ID NO: 30004 - DNA, 28 bp, synthetic construct
  source 1..28: mol_type = other DNA
gggcggcgcggcctgcgagcgccgcggg

SEQ ID NO: 30005 - DNA, 28 bp, synthetic construct
  source 1..28: mol_type = other DNA
agggcggcgcggcctgcgagcgccgcgg

SEQ ID NO: 30006 - DNA, 28 bp, synthetic construct
  source 1..28: mol_type = other DNA
acgagagaggggcggcagggcggcgcgg

SEQ ID NO: 30007 - DNA, 28 bp, synthetic construct
  source 1..28: mol_type = other DNA
gcgccgccctgccgcccctctctcgtgg

SEQ ID NO: 30008 - DNA, 28 bp, synthetic construct
  source 1..28: mol_type = other DNA
aagccacgagagaggggcggcagggcgg

SEQ ID NO: 30009 - DNA, 28 bp, synthetic construct
  source 1..28: mol_type = other DNA
taaaagccacgagagaggggcggcaggg

SEQ ID NO: 30010 - DNA, 28 bp, synthetic construct
  source 1..28: mol_type = other DNA
gtaaaagccacgagagaggggcggcagg

SEQ ID NO: 30011 - DNA, 28 bp, synthetic construct
  source 1..28: mol_type = other DNA
tgccgcccctctctcgtggcttttacgg

SEQ ID NO: 30012 - DNA, 28 bp, synthetic construct
  source 1..28: mol_type = other DNA
ggccgtaaaagccacgagagaggggcgg

SEQ ID NO: 30013 - DNA, 28 bp, synthetic construct
  source 1..28: mol_type = other DNA
gcgggccgtaaaagccacgagagagggg

SEQ ID NO: 30014 - DNA, 28 bp, synthetic construct
  source 1..28: mol_type = other DNA
ggcgggccgtaaaagccacgagagaggg

SEQ ID NO: 30015 - DNA, 28 bp, synthetic construct
  source 1..28: mol_type = other DNA
gggcgggccgtaaaagccacgagagagg

SEQ ID NO: 30016 - DNA, 28 bp, synthetic construct
  source 1..28: mol_type = other DNA
cggcccgcccgcccctcagcagccctgg

SEQ ID NO: 30017 - DNA, 28 bp, synthetic construct
  source 1..28: mol_type = other DNA
ggcccgcccgcccctcagcagccctggg

SEQ ID NO: 30018 - DNA, 28 bp, synthetic construct
  source 1..28: mol_type = other DNA
gcccgcccgcccctcagcagccctgggg

SEQ ID NO: 30019 - DNA, 28 bp, synthetic construct
  source 1..28: mol_type = other DNA
accccagggctgctgaggggcgggcggg

SEQ ID NO: 30020 - DNA, 28 bp, synthetic construct
  source 1..28: mol_type = other DNA
caccccagggctgctgaggggcgggcgg

SEQ ID NO: 30021 - DNA, 28 bp, synthetic construct
  source 1..28: mol_type = other DNA
gggcaccccagggctgctgaggggcggg

SEQ ID NO: 30022 - DNA, 28 bp, synthetic construct
  source 1..28: mol_type = other DNA
cgggcaccccagggctgctgaggggcgg

SEQ ID NO: 30023 - DNA, 28 bp, synthetic construct
  source 1..28: mol_type = other DNA
cgcccctcagcagccctggggtgcccgg

SEQ ID NO: 30024 - DNA, 28 bp, synthetic construct
  source 1..28: mol_type = other DNA
gcccctcagcagccctggggtgcccggg

SEQ ID NO: 30025 - DNA, 28 bp, synthetic construct
  source 1..28: mol_type = other DNA
cccctcagcagccctggggtgcccgggg

SEQ ID NO: 30026 - DNA, 28 bp, synthetic construct
  source 1..28: mol_type = other DNA
gccccgggcaccccagggctgctgaggg

SEQ ID NO: 30027 - DNA, 28 bp, synthetic construct
  source 1..28: mol_type = other DNA
cgccccgggcaccccagggctgctgagg

SEQ ID NO: 30028 - DNA, 28 bp, synthetic construct
  source 1..28: mol_type = other DNA
ctcagcagccctggggtgcccggggcgg

SEQ ID NO: 30029 - DNA, 28 bp, synthetic construct
  source 1..28: mol_type = other DNA
ttgcagggccgccccgggcaccccaggg

SEQ ID NO: 30030 - DNA, 28 bp, synthetic construct
  source 1..28: mol_type = other DNA
cttgcagggccgccccgggcaccccagg

SEQ ID NO: 30031 - DNA, 28 bp, synthetic construct
  source 1..28: mol_type = other DNA
ggggtgcccggggcggccctgcaagcgg

SEQ ID NO: 30032 - DNA, 28 bp, synthetic construct
  source 1..28: mol_type = other DNA
gggtgcccggggcggccctgcaagcggg

SEQ ID NO: 30033 - DNA, 28 bp, synthetic construct
  source 1..28: mol_type = other DNA
tctctcccgcttgcagggccgccccggg

SEQ ID NO: 30034 - DNA, 28 bp, synthetic construct
  source 1..28: mol_type = other DNA
ctctctcccgcttgcagggccgccccgg

SEQ ID NO: 30035 - DNA, 28 bp, synthetic construct
  source 1..28: mol_type = other DNA
gggcggccctgcaagcgggagagagcgg

SEQ ID NO: 30036 - DNA, 28 bp, synthetic construct
  source 1..28: mol_type = other DNA
gccctgcaagcgggagagagcggcgagg

SEQ ID NO: 30037 - DNA, 28 bp, synthetic construct
  source 1..28: mol_type = other DNA
gcctcgccgctctctcccgcttgcaggg

SEQ ID NO: 30038 - DNA, 28 bp, synthetic construct
  source 1..28: mol_type = other DNA
cgcctcgccgctctctcccgcttgcagg

SEQ ID NO: 30039 - DNA, 28 bp, synthetic construct
  source 1..28: mol_type = other DNA
ctgcaagcgggagagagcggcgaggcgg

SEQ ID NO: 30040 - DNA, 28 bp, synthetic construct
  source 1..28: mol_type = other DNA
caagcgggagagagcggcgaggcggcgg

SEQ ID NO: 30041 - DNA, 28 bp, synthetic construct
  source 1..28: mol_type = other DNA
agcggcgaggcggcggcgccgagtgcgg

SEQ ID NO: 30042 - DNA, 28 bp, synthetic construct
  source 1..28: mol_type = other DNA
gcggcgaggcggcggcgccgagtgcggg

SEQ ID NO: 30043 - DNA, 28 bp, synthetic construct
  source 1..28: mol_type = other DNA
cggcgaggcggcggcgccgagtgcgggg

SEQ ID NO: 30044 - DNA, 28 bp, synthetic construct
  source 1..28: mol_type = other DNA
ggcgaggcggcggcgccgagtgcggggg

SEQ ID NO: 30045 - DNA, 28 bp, synthetic construct
  source 1..28: mol_type = other DNA
gcgaggcggcggcgccgagtgcgggggg

SEQ ID NO: 30046 - DNA, 28 bp, synthetic construct
  source 1..28: mol_type = other DNA
cggcggcgccgagtgcggggggatgcgg

SEQ ID NO: 30047 - DNA, 28 bp, synthetic construct
  source 1..28: mol_type = other DNA
gcacggctccgcatccccccgcactcgg

SEQ ID NO: 30048 - DNA, 28 bp, synthetic construct
  source 1..28: mol_type = other DNA
gtgcggggggatgcggagccgtgcccgg

SEQ ID NO: 30049 - DNA, 28 bp, synthetic construct
  source 1..28: mol_type = other DNA
ccgagggatgcgacagggccgggcacgg

SEQ ID NO: 30050 - DNA, 28 bp, synthetic construct
  source 1..28: mol_type = other DNA
ggcggccgagggatgcgacagggccggg

SEQ ID NO: 30051 - DNA, 28 bp, synthetic construct
  source 1..28: mol_type = other DNA
gggcggccgagggatgcgacagggccgg

SEQ ID NO: 30052 - DNA, 28 bp, synthetic construct
  source 1..28: mol_type = other DNA
gggcgggcggccgagggatgcgacaggg

SEQ ID NO: 30053 - DNA, 28 bp, synthetic construct
  source 1..28: mol_type = other DNA
cgggcgggcggccgagggatgcgacagg

SEQ ID NO: 30054 - DNA, 28 bp, synthetic construct
  source 1..28: mol_type = other DNA
catccctcggccgcccgcccgcgcccgg

SEQ ID NO: 30055 - DNA, 28 bp, synthetic construct
  source 1..28: mol_type = other DNA
gggccgggcgcgggcgggcggccgaggg

SEQ ID NO: 30056 - DNA, 28 bp, synthetic construct
  source 1..28: mol_type = other DNA
ggggccgggcgcgggcgggcggccgagg

SEQ ID NO: 30057 - DNA, 28 bp, synthetic construct
  source 1..28: mol_type = other DNA
ccgcccgcccgcgcccggccccgcccgg

SEQ ID NO: 30058 - DNA, 28 bp, synthetic construct
  source 1..28: mol_type = other DNA
aggccgggcggggccgggcgcgggcggg

SEQ ID NO: 30059 - DNA, 28 bp, synthetic construct
  source 1..28: mol_type = other DNA
aaggccgggcggggccgggcgcgggcgg

SEQ ID NO: 30060 - DNA, 28 bp, synthetic construct
  source 1..28: mol_type = other DNA
ggcaaggccgggcggggccgggcgcggg

SEQ ID NO: 30061 - DNA, 28 bp, synthetic construct
  source 1..28: mol_type = other DNA
gggcaaggccgggcggggccgggcgcgg

SEQ ID NO: 30062 - DNA, 28 bp, synthetic construct
  source 1..28: mol_type = other DNA
gcgcccggccccgcccggccttgcccgg

SEQ ID NO: 30063 - DNA, 28 bp, synthetic construct
  source 1..28: mol_type = other DNA
cgcccggccccgcccggccttgcccggg

SEQ ID NO: 30064 - DNA, 28 bp, synthetic construct
  source 1..28: mol_type = other DNA
agcccgggcaaggccgggcggggccggg

SEQ ID NO: 30065 - DNA, 28 bp, synthetic construct
  source 1..28: mol_type = other DNA
cagcccgggcaaggccgggcggggccgg

SEQ ID NO: 30066 - DNA, 28 bp, synthetic construct
  source 1..28: mol_type = other DNA
cgtgcagcccgggcaaggccgggcgggg

SEQ ID NO: 30067 - DNA, 28 bp, synthetic construct
  source 1..28: mol_type = other DNA
gcgtgcagcccgggcaaggccgggcggg

SEQ ID NO: 30068 - DNA, 28 bp, synthetic construct
  source 1..28: mol_type = other DNA
tgcgtgcagcccgggcaaggccgggcgg

SEQ ID NO: 30069 - DNA, 28 bp, synthetic construct
  source 1..28: mol_type = other DNA
aagtgcgtgcagcccgggcaaggccggg

SEQ ID NO: 30070 - DNA, 28 bp, synthetic construct
  source 1..28: mol_type = other DNA
gaagtgcgtgcagcccgggcaaggccgg

SEQ ID NO: 30071 - DNA, 28 bp, synthetic construct
  source 1..28: mol_type = other DNA
gggagaagtgcgtgcagcccgggcaagg

SEQ ID NO: 30072 - DNA, 28 bp, synthetic construct
  source 1..28: mol_type = other DNA
gcccgggctgcacgcacttctcccgcgg

SEQ ID NO: 30073 - DNA, 28 bp, synthetic construct
  source 1..28: mol_type = other DNA
gccgcgggagaagtgcgtgcagcccggg

SEQ ID NO: 30074 - DNA, 28 bp, synthetic construct
  source 1..28: mol_type = other DNA
ggccgcgggagaagtgcgtgcagcccgg

SEQ ID NO: 30075 - DNA, 28 bp, synthetic construct
  source 1..28: mol_type = other DNA
cagggtcaagtggattctgggccgcggg

SEQ ID NO: 30076 - DNA, 28 bp, synthetic construct
  source 1..28: mol_type = other DNA
gcagggtcaagtggattctgggccgcgg

SEQ ID NO: 30077 - DNA, 28 bp, synthetic construct
  source 1..28: mol_type = other DNA
cggcccagaatccacttgaccctgctgg

SEQ ID NO: 30078 - DNA, 28 bp, synthetic construct
  source 1..28: mol_type = other DNA
ggcccagaatccacttgaccctgctggg

SEQ ID NO: 30079 - DNA, 28 bp, synthetic construct
  source 1..28: mol_type = other DNA
cgcccagcagggtcaagtggattctggg

SEQ ID NO: 30080 - DNA, 28 bp, synthetic construct
  source 1..28: mol_type = other DNA
gcgcccagcagggtcaagtggattctgg

SEQ ID NO: 30081 - DNA, 28 bp, synthetic construct
  source 1..28: mol_type = other DNA
cgcgggagcgcccagcagggtcaagtgg

SEQ ID NO: 30082 - DNA, 28 bp, synthetic construct
  source 1..28: mol_type = other DNA
cacttgaccctgctgggcgctcccgcgg

SEQ ID NO: 30083 - DNA, 28 bp, synthetic construct
  source 1..28: mol_type = other DNA
acttgaccctgctgggcgctcccgcggg

SEQ ID NO: 30084 - DNA, 28 bp, synthetic construct
  source 1..28: mol_type = other DNA
tgaccctgctgggcgctcccgcgggcgg

SEQ ID NO: 30085 - DNA, 28 bp, synthetic construct
  source 1..28: mol_type = other DNA
ccgccgcccgcgggagcgcccagcaggg

SEQ ID NO: 30086 - DNA, 28 bp, synthetic construct
  source 1..28: mol_type = other DNA
tccgccgcccgcgggagcgcccagcagg

SEQ ID NO: 30087 - DNA, 28 bp, synthetic construct
  source 1..28: mol_type = other DNA
tgggcgctcccgcgggcggcggacccgg

SEQ ID NO: 30088 - DNA, 28 bp, synthetic construct
  source 1..28: mol_type = other DNA
gggcgctcccgcgggcggcggacccggg

SEQ ID NO: 30089 - DNA, 28 bp, synthetic construct
  source 1..28: mol_type = other DNA
cgctcccgcgggcggcggacccgggtgg

SEQ ID NO: 30090 - DNA, 28 bp, synthetic construct
  source 1..28: mol_type = other DNA
gctcccgcgggcggcggacccgggtggg

SEQ ID NO: 30091 - DNA, 28 bp, synthetic construct
  source 1..28: mol_type = other DNA
gcacccacccgggtccgccgcccgcggg

SEQ ID NO: 30092 - DNA, 28 bp, synthetic construct
  source 1..28: mol_type = other DNA
cgcacccacccgggtccgccgcccgcgg

SEQ ID NO: 30093 - DNA, 28 bp, synthetic construct
  source 1..28: mol_type = other DNA
cgcgggcggcggacccgggtgggtgcgg

SEQ ID NO: 30094 - DNA, 28 bp, synthetic construct
  source 1..28: mol_type = other DNA
gcgggcggcggacccgggtgggtgcggg

SEQ ID NO: 30095 - DNA, 28 bp, synthetic construct
  source 1..28: mol_type = other DNA
cgggcggcggacccgggtgggtgcgggg

SEQ ID NO: 30096 - DNA, 28 bp, synthetic construct
  source 1..28: mol_type = other DNA
gggcggcggacccgggtgggtgcggggg

SEQ ID NO: 30097 - DNA, 28 bp, synthetic construct
  source 1..28: mol_type = other DNA
ccggggaattcccccgcacccacccggg

SEQ ID NO: 30098 - DNA, 28 bp, synthetic construct
  source 1..28: mol_type = other DNA
gccggggaattcccccgcacccacccgg

SEQ ID NO: 30099 - DNA, 28 bp, synthetic construct
  source 1..28: mol_type = other DNA
gtgcgggggaattccccggccgcccagg

SEQ ID NO: 30100 - DNA, 28 bp, synthetic construct
  source 1..28: mol_type = other DNA
ggggaattccccggccgcccaggcgcgg

SEQ ID NO: 30101 - DNA, 28 bp, synthetic construct
  source 1..28: mol_type = other DNA
gggaattccccggccgcccaggcgcggg

SEQ ID NO: 30102 - DNA, 28 bp, synthetic construct
  source 1..28: mol_type = other DNA
ggaattccccggccgcccaggcgcgggg

SEQ ID NO: 30103 - DNA, 28 bp, synthetic construct
  source 1..28: mol_type = other DNA
cactctccccgcgcctgggcggccgggg

SEQ ID NO: 30104 - DNA, 28 bp, synthetic construct
  source 1..28: mol_type = other DNA
tcactctccccgcgcctgggcggccggg

SEQ ID NO: 30105 - DNA, 28 bp, synthetic construct
  source 1..28: mol_type = other DNA
ctcactctccccgcgcctgggcggccgg

SEQ ID NO: 30106 - DNA, 28 bp, synthetic construct
  source 1..28: mol_type = other DNA
acagctcactctccccgcgcctgggcgg

SEQ ID NO: 30107 - DNA, 28 bp, synthetic construct
  source 1..28: mol_type = other DNA
ggcacagctcactctccccgcgcctggg

SEQ ID NO: 30108 - DNA, 28 bp, synthetic construct
  source 1..28: mol_type = other DNA
cggcacagctcactctccccgcgcctgg

SEQ ID NO: 30109 - DNA, 28 bp, synthetic construct
  source 1..28: mol_type = other DNA
ggtttgtttggggcgctgctgcgggcgg

SEQ ID NO: 30110 - DNA, 28 bp, synthetic construct
  source 1..28: mol_type = other DNA
aacggtttgtttggggcgctgctgcggg

SEQ ID NO: 30111 - DNA, 28 bp, synthetic construct
  source 1..28: mol_type = other DNA
aaacggtttgtttggggcgctgctgcgg

SEQ ID NO: 30112 - DNA, 28 bp, synthetic construct
  source 1..28: mol_type = other DNA
agcagcgccccaaacaaaccgtttaagg

SEQ ID NO: 30113 - DNA, 28 bp, synthetic construct
  source 1..28: mol_type = other DNA
ccccaaacaaaccgtttaaggtctctgg

SEQ ID NO: 30114 - DNA, 28 bp, synthetic construct
  source 1..28: mol_type = other DNA
tccagagaccttaaacggtttgtttggg

SEQ ID NO: 30115 - DNA, 28 bp, synthetic construct
  source 1..28: mol_type = other DNA
ctccagagaccttaaacggtttgtttgg

SEQ ID NO: 30116 - DNA, 28 bp, synthetic construct
  source 1..28: mol_type = other DNA
acttgcgggctccagagaccttaaacgg

SEQ ID NO: 30117 - DNA, 28 bp, synthetic construct
  source 1..28: mol_type = other DNA
agcccgcaagttcagcgaaataaagcgg

SEQ ID NO: 30118 - DNA, 28 bp, synthetic construct
  source 1..28: mol_type = other DNA
cgccgctttatttcgctgaacttgcggg

SEQ ID NO: 30119 - DNA, 28 bp, synthetic construct
  source 1..28: mol_type = other DNA
ccgccgctttatttcgctgaacttgcgg

SEQ ID NO: 30120 - DNA, 28 bp, synthetic construct
  source 1..28: mol_type = other DNA
agttcagcgaaataaagcggcggcgcgg

SEQ ID NO: 30121 - DNA, 28 bp, synthetic construct
  source 1..28: mol_type = other DNA
tcagcgaaataaagcggcggcgcggagg

SEQ ID NO: 30122 - DNA, 28 bp, synthetic construct
  source 1..28: mol_type = other DNA
cggcgcggaggaaacctcttccacccgg

SEQ ID NO: 30123 - DNA, 28 bp, synthetic construct
  source 1..28: mol_type = other DNA
aacggagagcaggtccgggtggaagagg

SEQ ID NO: 30124 - DNA, 28 bp, synthetic construct
  source 1..28: mol_type = other DNA
ttccacccggacctgctctccgttgcgg

SEQ ID NO: 30125 - DNA, 28 bp, synthetic construct
  source 1..28: mol_type = other DNA
aaccgcaacggagagcaggtccgggtgg

SEQ ID NO: 30126 - DNA, 28 bp, synthetic construct
  source 1..28: mol_type = other DNA
ccaaaccgcaacggagagcaggtccggg

SEQ ID NO: 30127 - DNA, 28 bp, synthetic construct
  source 1..28: mol_type = other DNA
gccaaaccgcaacggagagcaggtccgg

SEQ ID NO: 30128 - DNA, 28 bp, synthetic construct
  source 1..28: mol_type = other DNA
tggaggccaaaccgcaacggagagcagg

SEQ ID NO: 30129 - DNA, 28 bp, synthetic construct
  source 1..28: mol_type = other DNA
ctctccgttgcggtttggcctccagtgg

SEQ ID NO: 30130 - DNA, 28 bp, synthetic construct
  source 1..28: mol_type = other DNA
tccgttgcggtttggcctccagtggtgg

SEQ ID NO: 30131 - DNA, 28 bp, synthetic construct
  source 1..28: mol_type = other DNA
accaccactggaggccaaaccgcaacgg

SEQ ID NO: 30132 - DNA, 28 bp, synthetic construct
  source 1..28: mol_type = other DNA
agagggtgggtgggaccaccactggagg

SEQ ID NO: 30133 - DNA, 28 bp, synthetic construct
  source 1..28: mol_type = other DNA
gctagagggtgggtgggaccaccactgg

SEQ ID NO: 30134 - DNA, 28 bp, synthetic construct
  source 1..28: mol_type = other DNA
gtggtggtcccacccaccctctagctgg

SEQ ID NO: 30135 - DNA, 28 bp, synthetic construct
  source 1..28: mol_type = other DNA
agggctggccagctagagggtgggtggg

SEQ ID NO: 30136 - DNA, 28 bp, synthetic construct
  source 1..28: mol_type = other DNA
cagggctggccagctagagggtgggtgg

SEQ ID NO: 30137 - DNA, 28 bp, synthetic construct
  source 1..28: mol_type = other DNA
cacccaccctctagctggccagccctgg

SEQ ID NO: 30138 - DNA, 28 bp, synthetic construct
  source 1..28: mol_type = other DNA
ttccagggctggccagctagagggtggg

SEQ ID NO: 30139 - DNA, 28 bp, synthetic construct
  source 1..28: mol_type = other DNA
tttccagggctggccagctagagggtgg

SEQ ID NO: 30140 - DNA, 28 bp, synthetic construct
  source 1..28: mol_type = other DNA
tggtttccagggctggccagctagaggg

SEQ ID NO: 30141 - DNA, 28 bp, synthetic construct
  source 1..28: mol_type = other DNA
ttggtttccagggctggccagctagagg

SEQ ID NO: 30142 - DNA, 28 bp, synthetic construct
  source 1..28: mol_type = other DNA
aagaaaggaggttggtttccagggctgg

SEQ ID NO: 30143 - DNA, 28 bp, synthetic construct
  source 1..28: mol_type = other DNA
taaaaagaaaggaggttggtttccaggg

SEQ ID NO: 30144 - DNA, 28 bp, synthetic construct
  source 1..28: mol_type = other DNA
ataaaaagaaaggaggttggtttccagg

SEQ ID NO: 30145 - DNA, 28 bp, synthetic construct
  source 1..28: mol_type = other DNA
ggtgagaaataaaaagaaaggaggttgg

SEQ ID NO: 30146 - DNA, 28 bp, synthetic construct
  source 1..28: mol_type = other DNA
aacctcctttctttttatttctcaccgg

SEQ ID NO: 30147 - DNA, 28 bp, synthetic construct
  source 1..28: mol_type = other DNA
acctcctttctttttatttctcaccggg

SEQ ID NO: 30148 - DNA, 28 bp, synthetic construct
  source 1..28: mol_type = other DNA
tcccggtgagaaataaaaagaaaggagg

SEQ ID NO: 30149 - DNA, 28 bp, synthetic construct
  source 1..28: mol_type = other DNA
cctttctttttatttctcaccgggaagg

SEQ ID NO: 30150 - DNA, 28 bp, synthetic construct
  source 1..28: mol_type = other DNA
ctttctttttatttctcaccgggaaggg

SEQ ID NO: 30151 - DNA, 28 bp, synthetic construct
  source 1..28: mol_type = other DNA
tttctttttatttctcaccgggaagggg

SEQ ID NO: 30152 - DNA, 28 bp, synthetic construct
  source 1..28: mol_type = other DNA
ttctttttatttctcaccgggaaggggg

SEQ ID NO: 30153 - DNA, 28 bp, synthetic construct
  source 1..28: mol_type = other DNA
tttctcaccgggaagggggacaaactgg

SEQ ID NO: 30154 - DNA, 28 bp, synthetic construct
  source 1..28: mol_type = other DNA
ccagaggccagtttgtcccccttcccgg

SEQ ID NO: 30155 - DNA, 28 bp, synthetic construct
  source 1..28: mol_type = other DNA
cgggaagggggacaaactggcctctggg

SEQ ID NO: 30156 - DNA, 28 bp, synthetic construct
  source 1..28: mol_type = other DNA
cggcaagtttgaagtcgacacccagagg

SEQ ID NO: 30157 - DNA, 28 bp, synthetic construct
  source 1..28: mol_type = other DNA
cgacttcaaacttgccgcccgtctccgg

SEQ ID NO: 30158 - DNA, 28 bp, synthetic construct
  source 1..28: mol_type = other DNA
tcaaacttgccgcccgtctccggtctgg

SEQ ID NO: 30159 - DNA, 28 bp, synthetic construct
  source 1..28: mol_type = other DNA
cttgccgcccgtctccggtctggaaagg

SEQ ID NO: 30160 - DNA, 28 bp, synthetic construct
  source 1..28: mol_type = other DNA
cctgcctttccagaccggagacgggcgg

SEQ ID NO: 30161 - DNA, 28 bp, synthetic construct
  source 1..28: mol_type = other DNA
tcacctgcctttccagaccggagacggg

SEQ ID NO: 30162 - DNA, 28 bp, synthetic construct
  source 1..28: mol_type = other DNA
atcacctgcctttccagaccggagacgg

SEQ ID NO: 30163 - DNA, 28 bp, synthetic construct
  source 1..28: mol_type = other DNA
tagctgatcacctgcctttccagaccgg

SEQ ID NO: 30164 - DNA, 28 bp, synthetic construct
  source 1..28: mol_type = other DNA
ctggaaaggcaggtgatcagctagaagg

SEQ ID NO: 30165 - DNA, 28 bp, synthetic construct
  source 1..28: mol_type = other DNA
tggaaaggcaggtgatcagctagaaggg

SEQ ID NO: 30166 - DNA, 28 bp, synthetic construct
  source 1..28: mol_type = other DNA
tagaagggtgataagagtatcatcgtgg

SEQ ID NO: 30167 - DNA, 28 bp, synthetic construct
  source 1..28: mol_type = other DNA
atgagggagattattattactctttagg

SEQ ID NO: 30168 - DNA, 28 bp, synthetic construct
  source 1..28: mol_type = other DNA
gggggaagagctgtctttacaatgaggg

SEQ ID NO: 30169 - DNA, 28 bp, synthetic construct
  source 1..28: mol_type = other DNA
agggggaagagctgtctttacaatgagg

SEQ ID NO: 30170 - DNA, 28 bp, synthetic construct
  source 1..28: mol_type = other DNA
tcattgtaaagacagctcttccccctgg

SEQ ID NO: 30171 - DNA, 28 bp, synthetic construct
  source 1..28: mol_type = other DNA
agcatgtctaaaaaagtaagccaggggg

SEQ ID NO: 30172 - DNA, 28 bp, synthetic construct
  source 1..28: mol_type = other DNA
cagcatgtctaaaaaagtaagccagggg

SEQ ID NO: 30173 - DNA, 28 bp, synthetic construct
  source 1..28: mol_type = other DNA
tcagcatgtctaaaaaagtaagccaggg

SEQ ID NO: 30174 - DNA, 28 bp, synthetic construct
  source 1..28: mol_type = other DNA
ctcagcatgtctaaaaaagtaagccagg

SEQ ID NO: 30175 - DNA, 28 bp, synthetic construct
  source 1..28: mol_type = other DNA
atgctgagaagcgcatgtctccatcagg

SEQ ID NO: 30176 - DNA, 28 bp, synthetic construct
  source 1..28: mol_type = other DNA
tgctgagaagcgcatgtctccatcaggg

SEQ ID NO: 30177 - DNA, 28 bp, synthetic construct
  source 1..28: mol_type = other DNA
tggagaagcagaggtagggccctgatgg

SEQ ID NO: 30178 - DNA, 28 bp, synthetic construct
  source 1..28: mol_type = other DNA
ggccctacctctgcttctccacagttgg

SEQ ID NO: 30179 - DNA, 28 bp, synthetic construct
  source 1..28: mol_type = other DNA
ggccaactgtggagaagcagaggtaggg

SEQ ID NO: 30180 - DNA, 28 bp, synthetic construct
  source 1..28: mol_type = other DNA
aggccaactgtggagaagcagaggtagg

SEQ ID NO: 30181 - DNA, 28 bp, synthetic construct
  source 1..28: mol_type = other DNA
ttctaggccaactgtggagaagcagagg

SEQ ID NO: 30182 - DNA, 28 bp, synthetic construct
  source 1..28: mol_type = other DNA
tgcttctccacagttggcctagaaccgg

SEQ ID NO: 30183 - DNA, 28 bp, synthetic construct
  source 1..28: mol_type = other DNA
ggggcttccggttctaggccaactgtgg

SEQ ID NO: 30184 - DNA, 28 bp, synthetic construct
  source 1..28: mol_type = other DNA
tggcctagaaccggaagcccctccaagg

SEQ ID NO: 30185 - DNA, 28 bp, synthetic construct
  source 1..28: mol_type = other DNA
gggccttggaggggcttccggttctagg

SEQ ID NO: 30186 - DNA, 28 bp, synthetic construct
  source 1..28: mol_type = other DNA
agtcagggggccttggaggggcttccgg

SEQ ID NO: 30187 - DNA, 28 bp, synthetic construct
  source 1..28: mol_type = other DNA
tcaggagagtcagggggccttggagggg

SEQ ID NO: 30188 - DNA, 28 bp, synthetic construct
  source 1..28: mol_type = other DNA
gtcaggagagtcagggggccttggaggg

SEQ ID NO: 30189 - DNA, 28 bp, synthetic construct
  source 1..28: mol_type = other DNA
ggtcaggagagtcagggggccttggagg

SEQ ID NO: 30190 - DNA, 28 bp, synthetic construct
  source 1..28: mol_type = other DNA
agaggtcaggagagtcagggggccttgg

SEQ ID NO: 30191 - DNA, 28 bp, synthetic construct
  source 1..28: mol_type = other DNA
aggccccctgactctcctgacctcttgg

SEQ ID NO: 30192 - DNA, 28 bp, synthetic construct
  source 1..28: mol_type = other DNA
tggccaagaggtcaggagagtcaggggg

SEQ ID NO: 30193 - DNA, 28 bp, synthetic construct
  source 1..28: mol_type = other DNA
gtggccaagaggtcaggagagtcagggg

SEQ ID NO: 30194 - DNA, 28 bp, synthetic construct
  source 1..28: mol_type = other DNA
tgtggccaagaggtcaggagagtcaggg

SEQ ID NO: 30195 - DNA, 28 bp, synthetic construct
  source 1..28: mol_type = other DNA
ctgtggccaagaggtcaggagagtcagg

SEQ ID NO: 30196 - DNA, 28 bp, synthetic construct
  source 1..28: mol_type = other DNA
tctcctgacctcttggccacagctccgg

SEQ ID NO: 30197 - DNA, 28 bp, synthetic construct
  source 1..28: mol_type = other DNA
aatccggagctgtggccaagaggtcagg

SEQ ID NO: 30198 - DNA, 28 bp, synthetic construct
  source 1..28: mol_type = other DNA
gtgagaatccggagctgtggccaagagg

SEQ ID NO: 30199 - DNA, 28 bp, synthetic construct
  source 1..28: mol_type = other DNA
ttggccacagctccggattctcaccagg

SEQ ID NO: 30200 - DNA, 28 bp, synthetic construct
  source 1..28: mol_type = other DNA
tggccacagctccggattctcaccaggg

SEQ ID NO: 30201 - DNA, 28 bp, synthetic construct
  source 1..28: mol_type = other DNA
aatccctggtgagaatccggagctgtgg

SEQ ID NO: 30202 - DNA, 28 bp, synthetic construct
  source 1..28: mol_type = other DNA
ttctggggaatccctggtgagaatccgg

SEQ ID NO: 30203 - DNA, 28 bp, synthetic construct
  source 1..28: mol_type = other DNA
ctctctaggaattctggggaatccctgg

SEQ ID NO: 30204 - DNA, 28 bp, synthetic construct
  source 1..28: mol_type = other DNA
tctgagctgctctctaggaattctgggg

SEQ ID NO: 30205 - DNA, 28 bp, synthetic construct
  source 1..28: mol_type = other DNA
ctctgagctgctctctaggaattctggg

SEQ ID NO: 30206 - DNA, 28 bp, synthetic construct
  source 1..28: mol_type = other DNA
gctctgagctgctctctaggaattctgg

SEQ ID NO: 30207 - DNA, 28 bp, synthetic construct
  source 1..28: mol_type = other DNA
actgcagggctctgagctgctctctagg

SEQ ID NO: 30208 - DNA, 28 bp, synthetic construct
  source 1..28: mol_type = other DNA
gttcgcgtggtgaggcacaactgcaggg

SEQ ID NO: 30209 - DNA, 28 bp, synthetic construct
  source 1..28: mol_type = other DNA
ggttcgcgtggtgaggcacaactgcagg

SEQ ID NO: 30210 - DNA, 28 bp, synthetic construct
  source 1..28: mol_type = other DNA
agtgcgaggtttggttcgcgtggtgagg

SEQ ID NO: 30211 - DNA, 28 bp, synthetic construct
  source 1..28: mol_type = other DNA
cggggagtgcgaggtttggttcgcgtgg

SEQ ID NO: 30212 - DNA, 28 bp, synthetic construct
  source 1..28: mol_type = other DNA
accaaacctcgcactccccgccaaaagg

SEQ ID NO: 30213 - DNA, 28 bp, synthetic construct
  source 1..28: mol_type = other DNA
cccttttggcggggagtgcgaggtttgg

SEQ ID NO: 30214 - DNA, 28 bp, synthetic construct
  source 1..28: mol_type = other DNA
ggactcccttttggcggggagtgcgagg

SEQ ID NO: 30215 - DNA, 28 bp, synthetic construct
  source 1..28: mol_type = other DNA
tgctggaagggactcccttttggcgggg

SEQ ID NO: 30216 - DNA, 28 bp, synthetic construct
  source 1..28: mol_type = other DNA
gtgctggaagggactcccttttggcggg

SEQ ID NO: 30217 - DNA, 28 bp, synthetic construct
  source 1..28: mol_type = other DNA
agtgctggaagggactcccttttggcgg

SEQ ID NO: 30218 - DNA, 28 bp, synthetic construct
  source 1..28: mol_type = other DNA
gagagtgctggaagggactcccttttgg

SEQ ID NO: 30219 - DNA, 28 bp, synthetic construct
  source 1..28: mol_type = other DNA
aggaacaaaggggagagtgctggaaggg

SEQ ID NO: 30220 - DNA, 28 bp, synthetic construct
  source 1..28: mol_type = other DNA
aaggaacaaaggggagagtgctggaagg

SEQ ID NO: 30221 - DNA, 28 bp, synthetic construct
  source 1..28: mol_type = other DNA
gaaaaaggaacaaaggggagagtgctgg

SEQ ID NO: 30222 - DNA, 28 bp, synthetic construct
  source 1..28: mol_type = other DNA
gcactctcccctttgttcctttttctgg

SEQ ID NO: 30223 - DNA, 28 bp, synthetic construct
  source 1..28: mol_type = other DNA
cactctcccctttgttcctttttctggg

SEQ ID NO: 30224 - DNA, 28 bp, synthetic construct
  source 1..28: mol_type = other DNA
ttcttgcccagaaaaaggaacaaagggg

SEQ ID NO: 30225 - DNA, 28 bp, synthetic construct
  source 1..28: mol_type = other DNA
gttcttgcccagaaaaaggaacaaaggg

SEQ ID NO: 30226 - DNA, 28 bp, synthetic construct
  source 1..28: mol_type = other DNA
ggttcttgcccagaaaaaggaacaaagg

SEQ ID NO: 30227 - DNA, 28 bp, synthetic construct
  source 1..28: mol_type = other DNA
cagtcagcggttcttgcccagaaaaagg

SEQ ID NO: 30228 - DNA, 28 bp, synthetic construct
  source 1..28: mol_type = other DNA
ctttttctgggcaagaaccgctgactgg

SEQ ID NO: 30229 - DNA, 28 bp, synthetic construct
  source 1..28: mol_type = other DNA
tttttctgggcaagaaccgctgactggg

SEQ ID NO: 30230 - DNA, 28 bp, synthetic construct
  source 1..28: mol_type = other DNA
ttttctgggcaagaaccgctgactgggg

SEQ ID NO: 30231 - DNA, 28 bp, synthetic construct
  source 1..28: mol_type = other DNA
ttacatttctggcagccccagtcagcgg

SEQ ID NO: 30232 - DNA, 28 bp, synthetic construct
  source 1..28: mol_type = other DNA
ctggggctgccagaaatgtaaaccctgg

SEQ ID NO: 30233 - DNA, 28 bp, synthetic construct
  source 1..28: mol_type = other DNA
tggggctgccagaaatgtaaaccctggg

SEQ ID NO: 30234 - DNA, 28 bp, synthetic construct
  source 1..28: mol_type = other DNA
cacttgcacccagggtttacatttctgg

SEQ ID NO: 30235 - DNA, 28 bp, synthetic construct
  source 1..28: mol_type = other DNA
aaatgtaaaccctgggtgcaagtgacgg

SEQ ID NO: 30236 - DNA, 28 bp, synthetic construct
  source 1..28: mol_type = other DNA
aatgtaaaccctgggtgcaagtgacggg

SEQ ID NO: 30237 - DNA, 28 bp, synthetic construct
  source 1..28: mol_type = other DNA
ggagggatcccgtcacttgcacccaggg

SEQ ID NO: 30238 - DNA, 28 bp, synthetic construct
  source 1..28: mol_type = other DNA
tggagggatcccgtcacttgcacccagg

SEQ ID NO: 30239 - DNA, 28 bp, synthetic construct
  source 1..28: mol_type = other DNA
gatgactcttcggcttgacgctggaggg

SEQ ID NO: 30240 - DNA, 28 bp, synthetic construct
  source 1..28: mol_type = other DNA
ggatgactcttcggcttgacgctggagg

SEQ ID NO: 30241 - DNA, 28 bp, synthetic construct
  source 1..28: mol_type = other DNA
agaggatgactcttcggcttgacgctgg

SEQ ID NO: 30242 - DNA, 28 bp, synthetic construct
  source 1..28: mol_type = other DNA
tgggtgaggtgagaggatgactcttcgg

SEQ ID NO: 30243 - DNA, 28 bp, synthetic construct
  source 1..28: mol_type = other DNA
ctcattcggaggtgggtgaggtgagagg

SEQ ID NO: 30244 - DNA, 28 bp, synthetic construct
  source 1..28: mol_type = other DNA
ctctcacctcacccacctccgaatgagg

SEQ ID NO: 30245 - DNA, 28 bp, synthetic construct
  source 1..28: mol_type = other DNA
gttaatcctcattcggaggtgggtgagg

SEQ ID NO: 30246 - DNA, 28 bp, synthetic construct
  source 1..28: mol_type = other DNA
agtttgttaatcctcattcggaggtggg

SEQ ID NO: 30247 - DNA, 28 bp, synthetic construct
  source 1..28: mol_type = other DNA
gagtttgttaatcctcattcggaggtgg

SEQ ID NO: 30248 - DNA, 28 bp, synthetic construct
  source 1..28: mol_type = other DNA
attgagtttgttaatcctcattcggagg

SEQ ID NO: 30249 - DNA, 28 bp, synthetic construct
  source 1..28: mol_type = other DNA
tgaattgagtttgttaatcctcattcgg

SEQ ID NO: 30250 - DNA, 28 bp, synthetic construct
  source 1..28: mol_type = other DNA
gaatgaggattaacaaactcaattcagg

SEQ ID NO: 30251 - DNA, 28 bp, synthetic construct
  source 1..28: mol_type = other DNA
gattaacaaactcaattcaggacacagg

SEQ ID NO: 30252 - DNA, 28 bp, synthetic construct
  source 1..28: mol_type = other DNA
ttcaggacacaggtagaagaccaaaagg

SEQ ID NO: 30253 - DNA, 28 bp, synthetic construct
  source 1..28: mol_type = other DNA
taggaaagaagtctcattggccttttgg

SEQ ID NO: 30254 - DNA, 28 bp, synthetic construct
  source 1..28: mol_type = other DNA
atctcaaataggaaagaagtctcattgg

SEQ ID NO: 30255 - DNA, 28 bp, synthetic construct
  source 1..28: mol_type = other DNA
atgagacttctttcctatttgagatcgg

SEQ ID NO: 30256 - DNA, 28 bp, synthetic construct
  source 1..28: mol_type = other DNA
agcattctcaaatccgatctcaaatagg

SEQ ID NO: 30257 - DNA, 28 bp, synthetic construct
  source 1..28: mol_type = other DNA
agatcggatttgagaatgctcagcctgg

SEQ ID NO: 30258 - DNA, 28 bp, synthetic construct
  source 1..28: mol_type = other DNA
tcagagctgggggaagaagggagccagg

SEQ ID NO: 30259 - DNA, 28 bp, synthetic construct
  source 1..28: mol_type = other DNA
gattgattcagagctgggggaagaaggg

SEQ ID NO: 30260 - DNA, 28 bp, synthetic construct
  source 1..28: mol_type = other DNA
ggattgattcagagctgggggaagaagg

SEQ ID NO: 30261 - DNA, 28 bp, synthetic construct
  source 1..28: mol_type = other DNA
gaagaaaggattgattcagagctggggg

SEQ ID NO: 30262 - DNA, 28 bp, synthetic construct
  source 1..28: mol_type = other DNA
tgaagaaaggattgattcagagctgggg

SEQ ID NO: 30263 - DNA, 28 bp, synthetic construct
  source 1..28: mol_type = other DNA
atgaagaaaggattgattcagagctggg

SEQ ID NO: 30264 - DNA, 28 bp, synthetic construct
  source 1..28: mol_type = other DNA
aatgaagaaaggattgattcagagctgg

SEQ ID NO: 30265 - DNA, 28 bp, synthetic construct
  source 1..28: mol_type = other DNA
attagttatggatgctaatgaagaaagg

SEQ ID NO: 30266 - DNA, 28 bp, synthetic construct
  source 1..28: mol_type = other DNA
cgttttacattttgcacattagttatgg

SEQ ID NO: 30267 - DNA, 28 bp, synthetic construct
  source 1..28: mol_type = other DNA
gtaaaacgctaaattaagacagagttgg

SEQ ID NO: 30268 - DNA, 28 bp, synthetic construct
  source 1..28: mol_type = other DNA
ttcagctaatgagaggggtttttgaggg

SEQ ID NO: 30269 - DNA, 28 bp, synthetic construct
  source 1..28: mol_type = other DNA
cttcagctaatgagaggggtttttgagg

SEQ ID NO: 30270 - DNA, 28 bp, synthetic construct
  source 1..28: mol_type = other DNA
ctcaaaaacccctctcattagctgaagg

SEQ ID NO: 30271 - DNA, 28 bp, synthetic construct
  source 1..28: mol_type = other DNA
acttgctaccttcagctaatgagagggg

SEQ ID NO: 30272 - DNA, 28 bp, synthetic construct
  source 1..28: mol_type = other DNA
tacttgctaccttcagctaatgagaggg

SEQ ID NO: 30273 - DNA, 28 bp, synthetic construct
  source 1..28: mol_type = other DNA
ctacttgctaccttcagctaatgagagg

SEQ ID NO: 30274 - DNA, 28 bp, synthetic construct
  source 1..28: mol_type = other DNA
gaaggtagcaagtagcaagaagattagg

SEQ ID NO: 30275 - DNA, 28 bp, synthetic construct
  source 1..28: mol_type = other DNA
gtaaaaacatagagaatatgaatatagg

SEQ ID NO: 30276 - DNA, 28 bp, synthetic construct
  source 1..28: mol_type = other DNA
agaatatgaatataggaaaaagtacagg

SEQ ID NO: 30277 - DNA, 28 bp, synthetic construct
  source 1..28: mol_type = other DNA
aatataggaaaaagtacaggtgtgaagg

SEQ ID NO: 30278 - DNA, 28 bp, synthetic construct
  source 1..28: mol_type = other DNA
atataggaaaaagtacaggtgtgaaggg

SEQ ID NO: 30279 - DNA, 28 bp, synthetic construct
  source 1..28: mol_type = other DNA
aggaaaaagtacaggtgtgaagggctgg

SEQ ID NO: 30280 - DNA, 28 bp, synthetic construct
  source 1..28: mol_type = other DNA
cccaaatcccaatgcacagtgtatttgg

SEQ ID NO: 30281 - DNA, 28 bp, synthetic construct
  source 1..28: mol_type = other DNA
tccaaatacactgtgcattgggatttgg

SEQ ID NO: 30282 - DNA, 28 bp, synthetic construct
  source 1..28: mol_type = other DNA
tctttttccaaatacactgtgcattggg

SEQ ID NO: 30283 - DNA, 28 bp, synthetic construct
  source 1..28: mol_type = other DNA
ttctttttccaaatacactgtgcattgg

SEQ ID NO: 30284 - DNA, 28 bp, synthetic construct
  source 1..28: mol_type = other DNA
aatatccccttagcatacgccttgttgg

SEQ ID NO: 30285 - DNA, 28 bp, synthetic construct
  source 1..28: mol_type = other DNA
catttccaacaaggcgtatgctaagggg

SEQ ID NO: 30286 - DNA, 28 bp, synthetic construct
  source 1..28: mol_type = other DNA
acatttccaacaaggcgtatgctaaggg

SEQ ID NO: 30287 - DNA, 28 bp, synthetic construct
  source 1..28: mol_type = other DNA
aacatttccaacaaggcgtatgctaagg

SEQ ID NO: 30288 - DNA, 28 bp, synthetic construct
  source 1..28: mol_type = other DNA
tacgccttgttggaaatgtttgctttgg

SEQ ID NO: 30289 - DNA, 28 bp, synthetic construct
  source 1..28: mol_type = other DNA
ttcgccaaagcaaacatttccaacaagg

SEQ ID NO: 30290 - DNA, 28 bp, synthetic construct
  source 1..28: mol_type = other DNA
atcgagacattgagacagcattcccagg

SEQ ID NO: 30291 - DNA, 28 bp, synthetic construct
  source 1..28: mol_type = other DNA
attgagacagcattcccaggaacaaagg

SEQ ID NO: 30292 - DNA, 28 bp, synthetic construct
  source 1..28: mol_type = other DNA
agacagcattcccaggaacaaaggctgg

SEQ ID NO: 30293 - DNA, 28 bp, synthetic construct
  source 1..28: mol_type = other DNA
gacagcattcccaggaacaaaggctggg

SEQ ID NO: 30294 - DNA, 28 bp, synthetic construct
  source 1..28: mol_type = other DNA
acagcattcccaggaacaaaggctgggg

SEQ ID NO: 30295 - DNA, 28 bp, synthetic construct
  source 1..28: mol_type = other DNA
cagcattcccaggaacaaaggctggggg

SEQ ID NO: 30296 - DNA, 28 bp, synthetic construct
  source 1..28: mol_type = other DNA
cattcccaggaacaaaggctgggggtgg

SEQ ID NO: 30297 - DNA, 28 bp, synthetic construct
  source 1..28: mol_type = other DNA
tcccaggaacaaaggctgggggtggagg

SEQ ID NO: 30298 - DNA, 28 bp, synthetic construct
  source 1..28: mol_type = other DNA
ccctccacccccagcctttgttcctggg

SEQ ID NO: 30299 - DNA, 28 bp, synthetic construct
  source 1..28: mol_type = other DNA
accctccacccccagcctttgttcctgg

SEQ ID NO: 30300 - DNA, 28 bp, synthetic construct
  source 1..28: mol_type = other DNA
aggaacaaaggctgggggtggagggtgg

SEQ ID NO: 30301 - DNA, 28 bp, synthetic construct
  source 1..28: mol_type = other DNA
aacaaaggctgggggtggagggtggagg

SEQ ID NO: 30302 - DNA, 28 bp, synthetic construct
  source 1..28: mol_type = other DNA
aaaggctgggggtggagggtggaggagg

SEQ ID NO: 30303 - DNA, 28 bp, synthetic construct
  source 1..28: mol_type = other DNA
aaggctgggggtggagggtggaggaggg

SEQ ID NO: 30304 - DNA, 28 bp, synthetic construct
  source 1..28: mol_type = other DNA
gggggtggagggtggaggagggagcagg

SEQ ID NO: 30305 - DNA, 28 bp, synthetic construct
  source 1..28: mol_type = other DNA
ggagggagcaggaacagcccctgtctgg

SEQ ID NO: 30306 - DNA, 28 bp, synthetic construct
  source 1..28: mol_type = other DNA
cagaacttgcagttcttccagacagggg

SEQ ID NO: 30307 - DNA, 28 bp, synthetic construct
  source 1..28: mol_type = other DNA
tcagaacttgcagttcttccagacaggg

SEQ ID NO: 30308 - DNA, 28 bp, synthetic construct
  source 1..28: mol_type = other DNA
ctcagaacttgcagttcttccagacagg

SEQ ID NO: 30309 - DNA, 28 bp, synthetic construct
  source 1..28: mol_type = other DNA
ctgtctggaagaactgcaagttctgagg

SEQ ID NO: 30310 - DNA, 28 bp, synthetic construct
  source 1..28: mol_type = other DNA
cgggaacaggacacatttcttgttcagg

SEQ ID NO: 30311 - DNA, 28 bp, synthetic construct
  source 1..28: mol_type = other DNA
gaaatgtgtcctgttcccgtgctcctgg

SEQ ID NO: 30312 - DNA, 28 bp, synthetic construct
  source 1..28: mol_type = other DNA
cagctgcagccaggagcacgggaacagg

SEQ ID NO: 30313 - DNA, 28 bp, synthetic construct
  source 1..28: mol_type = other DNA
ctgttcccgtgctcctggctgcagctgg

SEQ ID NO: 30314 - DNA, 28 bp, synthetic construct
  source 1..28: mol_type = other DNA
tgttcccgtgctcctggctgcagctggg

SEQ ID NO: 30315 - DNA, 28 bp, synthetic construct
  source 1..28: mol_type = other DNA
gcttcccagctgcagccaggagcacggg

SEQ ID NO: 30316 - DNA, 28 bp, synthetic construct
  source 1..28: mol_type = other DNA
agcttcccagctgcagccaggagcacgg

SEQ ID NO: 30317 - DNA, 28 bp, synthetic construct
  source 1..28: mol_type = other DNA
ctgaagaagcttcccagctgcagccagg

SEQ ID NO: 30318 - DNA, 28 bp, synthetic construct
  source 1..28: mol_type = other DNA
ctgcagctgggaagcttcttcagaaagg

SEQ ID NO: 30319 - DNA, 28 bp, synthetic construct
  source 1..28: mol_type = other DNA
aagcttcttcagaaaggagacctcccgg

SEQ ID NO: 30320 - DNA, 28 bp, synthetic construct
  source 1..28: mol_type = other DNA
agaaaggagacctcccggccctcaccgg

SEQ ID NO: 30321 - DNA, 28 bp, synthetic construct
  source 1..28: mol_type = other DNA
gaaaggagacctcccggccctcaccggg

SEQ ID NO: 30322 - DNA, 28 bp, synthetic construct
  source 1..28: mol_type = other DNA
agacctcccggccctcaccgggatctgg

SEQ ID NO: 30323 - DNA, 28 bp, synthetic construct
  source 1..28: mol_type = other DNA
aagccagatcccggtgagggccgggagg

SEQ ID NO: 30324 - DNA, 28 bp, synthetic construct
  source 1..28: mol_type = other DNA
ggaaagccagatcccggtgagggccggg

SEQ ID NO: 30325 - DNA, 28 bp, synthetic construct
  source 1..28: mol_type = other DNA
aggaaagccagatcccggtgagggccgg

SEQ ID NO: 30326 - DNA, 28 bp, synthetic construct
  source 1..28: mol_type = other DNA
gggaaggaaagccagatcccggtgaggg

SEQ ID NO: 30327 - DNA, 28 bp, synthetic construct
  source 1..28: mol_type = other DNA
agggaaggaaagccagatcccggtgagg

SEQ ID NO: 30328 - DNA, 28 bp, synthetic construct
  source 1..28: mol_type = other DNA
tgggaagggaaggaaagccagatcccgg

SEQ ID NO: 30329 - DNA, 28 bp, synthetic construct
  source 1..28: mol_type = other DNA
tataaacagatgtggtgggaagggaagg

SEQ ID NO: 30330 - DNA, 28 bp, synthetic construct
  source 1..28: mol_type = other DNA
tttgtataaacagatgtggtgggaaggg

SEQ ID NO: 30331 - DNA, 28 bp, synthetic construct
  source 1..28: mol_type = other DNA
ctttgtataaacagatgtggtgggaagg

SEQ ID NO: 30332 - DNA, 28 bp, synthetic construct
  source 1..28: mol_type = other DNA
cttcccaccacatctgtttatacaaagg

SEQ ID NO: 30333 - DNA, 28 bp, synthetic construct
  source 1..28: mol_type = other DNA
cccaccacatctgtttatacaaaggagg

SEQ ID NO: 30334 - DNA, 28 bp, synthetic construct
  source 1..28: mol_type = other DNA
ccctcctttgtataaacagatgtggtgg

SEQ ID NO: 30335 - DNA, 28 bp, synthetic construct
  source 1..28: mol_type = other DNA
cggccctcctttgtataaacagatgtgg

SEQ ID NO: 30336 - DNA, 28 bp, synthetic construct
  source 1..28: mol_type = other DNA
tgtttatacaaaggagggccgctgaagg

SEQ ID NO: 30337 - DNA, 28 bp, synthetic construct
  source 1..28: mol_type = other DNA
aaacacggttatgtttgtccttcagcgg

SEQ ID NO: 30338 - DNA, 28 bp, synthetic construct
  source 1..28: mol_type = other DNA
accgtgtttactgcgagtcccatgctgg

SEQ ID NO: 30339 - DNA, 28 bp, synthetic construct
  source 1..28: mol_type = other DNA
ccgtgtttactgcgagtcccatgctggg

SEQ ID NO: 30340 - DNA, 28 bp, synthetic construct
  source 1..28: mol_type = other DNA
tttactgcgagtcccatgctgggcctgg

SEQ ID NO: 30341 - DNA, 28 bp, synthetic construct
  source 1..28: mol_type = other DNA
tgtatctgagctccaggcccagcatggg

SEQ ID NO: 30342 - DNA, 28 bp, synthetic construct
  source 1..28: mol_type = other DNA
ctgtatctgagctccaggcccagcatgg

SEQ ID NO: 30343 - DNA, 28 bp, synthetic construct
  source 1..28: mol_type = other DNA
gagggcaaatctgtatctgagctccagg

SEQ ID NO: 30344 - DNA, 28 bp, synthetic construct
  source 1..28: mol_type = other DNA
ctcagatacagatttgccctcaccatgg

SEQ ID NO: 30345 - DNA, 28 bp, synthetic construct
  source 1..28: mol_type = other DNA
agatacagatttgccctcaccatggagg

SEQ ID NO: 30346 - DNA, 28 bp, synthetic construct
  source 1..28: mol_type = other DNA
tatttatcttcagcctccatggtgaggg

SEQ ID NO: 30347 - DNA, 28 bp, synthetic construct
  source 1..28: mol_type = other DNA
ctatttatcttcagcctccatggtgagg

SEQ ID NO: 30348 - DNA, 28 bp, synthetic construct
  source 1..28: mol_type = other DNA
atcatctatttatcttcagcctccatgg

SEQ ID NO: 30349 - DNA, 28 bp, synthetic construct
  source 1..28: mol_type = other DNA
gaagataaatagatgatcccagaaaagg

SEQ ID NO: 30350 - DNA, 28 bp, synthetic construct
  source 1..28: mol_type = other DNA
aatagatgatcccagaaaaggaaagagg

SEQ ID NO: 30351 - DNA, 28 bp, synthetic construct
  source 1..28: mol_type = other DNA
atagatgatcccagaaaaggaaagaggg

SEQ ID NO: 30352 - DNA, 28 bp, synthetic construct
  source 1..28: mol_type = other DNA
atgatcccagaaaaggaaagagggaagg

SEQ ID NO: 30353 - DNA, 28 bp, synthetic construct
  source 1..28: mol_type = other DNA
cagggccttccctctttccttttctggg

SEQ ID NO: 30354 - DNA, 28 bp, synthetic construct
  source 1..28: mol_type = other DNA
ccagaaaaggaaagagggaaggccctgg

SEQ ID NO: 30355 - DNA, 28 bp, synthetic construct
  source 1..28: mol_type = other DNA
cagaaaaggaaagagggaaggccctggg

SEQ ID NO: 30356 - DNA, 28 bp, synthetic construct
  source 1..28: mol_type = other DNA
aaaggaaagagggaaggccctgggatgg

SEQ ID NO: 30357 - DNA, 28 bp, synthetic construct
  source 1..28: mol_type = other DNA
ggaaggccctgggatggtatagagctgg

SEQ ID NO: 30358 - DNA, 28 bp, synthetic construct
  source 1..28: mol_type = other DNA
ccctgggatggtatagagctggttgagg

SEQ ID NO: 30359 - DNA, 28 bp, synthetic construct
  source 1..28: mol_type = other DNA
cctgggatggtatagagctggttgaggg

SEQ ID NO: 30360 - DNA, 28 bp, synthetic construct
  source 1..28: mol_type = other DNA
ctgggatggtatagagctggttgagggg

SEQ ID NO: 30361 - DNA, 28 bp, synthetic construct
  source 1..28: mol_type = other DNA
gctggttgaggggtttactcatgaaagg

SEQ ID NO: 30362 - DNA, 28 bp, synthetic construct
  source 1..28: mol_type = other DNA
cctctcccaaaaagccatgtagtaacgg

SEQ ID NO: 30363 - DNA, 28 bp, synthetic construct
  source 1..28: mol_type = other DNA
ctctcccaaaaagccatgtagtaacggg

SEQ ID NO: 30364 - DNA, 28 bp, synthetic construct
  source 1..28: mol_type = other DNA
tctgcccgttactacatggctttttggg

SEQ ID NO: 30365 - DNA, 28 bp, synthetic construct
  source 1..28: mol_type = other DNA
atctgcccgttactacatggctttttgg

SEQ ID NO: 30366 - DNA, 28 bp, synthetic construct
  source 1..28: mol_type = other DNA
aaacgtaaatctgcccgttactacatgg

SEQ ID NO: 30367 - DNA, 28 bp, synthetic construct
  source 1..28: mol_type = other DNA
cagatttacgtttgaatttaaactctgg

SEQ ID NO: 30368 - DNA, 28 bp, synthetic construct
  source 1..28: mol_type = other DNA
gcacacactctcatatattaacacaagg

SEQ ID NO: 30369 - DNA, 28 bp, synthetic construct
  source 1..28: mol_type = other DNA
agtgtgtgcacctaaagcaattgcaagg

SEQ ID NO: 30370 - DNA, 28 bp, synthetic construct
  source 1..28: mol_type = other DNA
gtgtgcacctaaagcaattgcaaggcgg

SEQ ID NO: 30371 - DNA, 28 bp, synthetic construct
  source 1..28: mol_type = other DNA
tgtgcacctaaagcaattgcaaggcggg

SEQ ID NO: 30372 - DNA, 28 bp, synthetic construct
  source 1..28: mol_type = other DNA
taaatacccgccttgcaattgctttagg

SEQ ID NO: 30373 - DNA, 28 bp, synthetic construct
  source 1..28: mol_type = other DNA
ggcgggtatttaaaaatgtttctttagg

SEQ ID NO: 30374 - DNA, 28 bp, synthetic construct
  source 1..28: mol_type = other DNA
ttaggaatagccatgattttctgtttgg

SEQ ID NO: 30375 - DNA, 28 bp, synthetic construct
  source 1..28: mol_type = other DNA
taggaatagccatgattttctgtttggg

SEQ ID NO: 30376 - DNA, 28 bp, synthetic construct
  source 1..28: mol_type = other DNA
aggaatagccatgattttctgtttgggg

SEQ ID NO: 30377 - DNA, 28 bp, synthetic construct
  source 1..28: mol_type = other DNA
gttagaggccccaaacagaaaatcatgg

SEQ ID NO: 30378 - DNA, 28 bp, synthetic construct
  source 1..28: mol_type = other DNA
gattttctgtttggggcctctaacatgg

SEQ ID NO: 30379 - DNA, 28 bp, synthetic construct
  source 1..28: mol_type = other DNA
attttctgtttggggcctctaacatggg

SEQ ID NO: 30380 - DNA, 28 bp, synthetic construct
  source 1..28: mol_type = other DNA
ttttctgtttggggcctctaacatgggg

SEQ ID NO: 30381 - DNA, 28 bp, synthetic construct
  source 1..28: mol_type = other DNA
ttggggcctctaacatggggatagttgg

SEQ ID NO: 30382 - DNA, 28 bp, synthetic construct
  source 1..28: mol_type = other DNA
atcaatccaactatccccatgttagagg

SEQ ID NO: 30383 - DNA, 28 bp, synthetic construct
  source 1..28: mol_type = other DNA
acactattacatgaaaacataacactgg

SEQ ID NO: 30384 - DNA, 28 bp, synthetic construct
  source 1..28: mol_type = other DNA
gttatgttttcatgtaatagtgtcttgg

SEQ ID NO: 30385 - DNA, 28 bp, synthetic construct
  source 1..28: mol_type = other DNA
tcatgtaatagtgtcttggagaatgagg

SEQ ID NO: 30386 - DNA, 28 bp, synthetic construct
  source 1..28: mol_type = other DNA
gtgtcttggagaatgaggacttttgagg

SEQ ID NO: 30387 - DNA, 28 bp, synthetic construct
  source 1..28: mol_type = other DNA
aaaacaggatctgcaactactatttggg

SEQ ID NO: 30388 - DNA, 28 bp, synthetic construct
  source 1..28: mol_type = other DNA
aaaaacaggatctgcaactactatttgg

SEQ ID NO: 30389 - DNA, 28 bp, synthetic construct
  source 1..28: mol_type = other DNA
gatcctgttttttactaagctgtcatgg

SEQ ID NO: 30390 - DNA, 28 bp, synthetic construct
  source 1..28: mol_type = other DNA
tctccatgacagcttagtaaaaaacagg

SEQ ID NO: 30391 - DNA, 28 bp, synthetic construct
  source 1..28: mol_type = other DNA
tacattttacttgtaaaaactattttgg

SEQ ID NO: 30392 - DNA, 28 bp, synthetic construct
  source 1..28: mol_type = other DNA
gtagaacagttagtgagagcctttatgg

SEQ ID NO: 30393 - DNA, 28 bp, synthetic construct
  source 1..28: mol_type = other DNA
tagaacagttagtgagagcctttatggg

SEQ ID NO: 30394 - DNA, 28 bp, synthetic construct
  source 1..28: mol_type = other DNA
gataaataataaagatctcccataaagg

SEQ ID NO: 30395 - DNA, 28 bp, synthetic construct
  source 1..28: mol_type = other DNA
ttatgggagatctttattatttatctgg

SEQ ID NO: 30396 - DNA, 28 bp, synthetic construct
  source 1..28: mol_type = other DNA
gatgttcctattatcctccagcctctgg

SEQ ID NO: 30397 - DNA, 28 bp, synthetic construct
  source 1..28: mol_type = other DNA
atgttcctattatcctccagcctctggg

SEQ ID NO: 30398 - DNA, 28 bp, synthetic construct
  source 1..28: mol_type = other DNA
gcatacccagaggctggaggataatagg

SEQ ID NO: 30399 - DNA, 28 bp, synthetic construct
  source 1..28: mol_type = other DNA
tttggtttgcatacccagaggctggagg

SEQ ID NO: 30400 - DNA, 28 bp, synthetic construct
  source 1..28: mol_type = other DNA
tgttttggtttgcatacccagaggctgg

SEQ ID NO: 30401 - DNA, 28 bp, synthetic construct
  source 1..28: mol_type = other DNA
tgcttgttttggtttgcatacccagagg

SEQ ID NO: 30402 - DNA, 28 bp, synthetic construct
  source 1..28: mol_type = other DNA
tgacaactagattaagtgcttgttttgg

SEQ ID NO: 30403 - DNA, 28 bp, synthetic construct
  source 1..28: mol_type = other DNA
taactccttaatacaaagcaaaaaaagg

SEQ ID NO: 30404 - DNA, 28 bp, synthetic construct
  source 1..28: mol_type = other DNA
aactccttaatacaaagcaaaaaaaggg

SEQ ID NO: 30405 - DNA, 28 bp, synthetic construct
  source 1..28: mol_type = other DNA
caaaccctttttttgctttgtattaagg

SEQ ID NO: 30406 - DNA, 28 bp, synthetic construct
  source 1..28: mol_type = other DNA
cttaatacaaagcaaaaaaagggtttgg

SEQ ID NO: 30407 - DNA, 28 bp, synthetic construct
  source 1..28: mol_type = other DNA
aaagcaaaaaaagggtttggacttttgg

SEQ ID NO: 30408 - DNA, 28 bp, synthetic construct
  source 1..28: mol_type = other DNA
aagcaaaaaaagggtttggacttttggg

SEQ ID NO: 30409 - DNA, 28 bp, synthetic construct
  source 1..28: mol_type = other DNA
agcaaaaaaagggtttggacttttgggg

SEQ ID NO: 30410 - DNA, 28 bp, synthetic construct
  source 1..28: mol_type = other DNA
tggggattagaatgtcagaactaaaagg

SEQ ID NO: 30411 - DNA, 28 bp, synthetic construct
  source 1..28: mol_type = other DNA
ggggattagaatgtcagaactaaaaggg

SEQ ID NO: 30412 - DNA, 28 bp, synthetic construct
  source 1..28: mol_type = other DNA
agcactataggatgagcaaaagctaagg

SEQ ID NO: 30413 - DNA, 28 bp, synthetic construct
  source 1..28: mol_type = other DNA
ctcatcctatagtgcttgtgacctgagg

SEQ ID NO: 30414 - DNA, 28 bp, synthetic construct
  source 1..28: mol_type = other DNA
tcatcctatagtgcttgtgacctgaggg

SEQ ID NO: 30415 - DNA, 28 bp, synthetic construct
  source 1..28: mol_type = other DNA
aagaccctcaggtcacaagcactatagg

SEQ ID NO: 30416 - DNA, 28 bp, synthetic construct
  source 1..28: mol_type = other DNA
gacctgagggtcttttctccccacatgg

SEQ ID NO: 30417 - DNA, 28 bp, synthetic construct
  source 1..28: mol_type = other DNA
atccatgtggggagaaaagaccctcagg

SEQ ID NO: 30418 - DNA, 28 bp, synthetic construct
  source 1..28: mol_type = other DNA
caggggtgttgcttgcatccatgtgggg

SEQ ID NO: 30419 - DNA, 28 bp, synthetic construct
  source 1..28: mol_type = other DNA
ccaggggtgttgcttgcatccatgtggg

SEQ ID NO: 30420 - DNA, 28 bp, synthetic construct
  source 1..28: mol_type = other DNA
ccacatggatgcaagcaacacccctggg

SEQ ID NO: 30421 - DNA, 28 bp, synthetic construct
  source 1..28: mol_type = other DNA
ctgggtggtttgattcagctcccagggg

SEQ ID NO: 30422 - DNA, 28 bp, synthetic construct
  source 1..28: mol_type = other DNA
gctgggtggtttgattcagctcccaggg

SEQ ID NO: 30423 - DNA, 28 bp, synthetic construct
  source 1..28: mol_type = other DNA
agctgggtggtttgattcagctcccagg

SEQ ID NO: 30424 - DNA, 28 bp, synthetic construct
  source 1..28: mol_type = other DNA
ggagctgaatcaaaccacccagctaagg

SEQ ID NO: 30425 - DNA, 28 bp, synthetic construct
  source 1..28: mol_type = other DNA
gagctgaatcaaaccacccagctaaggg

SEQ ID NO: 30426 - DNA, 28 bp, synthetic construct
  source 1..28: mol_type = other DNA
agctgaatcaaaccacccagctaagggg

SEQ ID NO: 30427 - DNA, 28 bp, synthetic construct
  source 1..28: mol_type = other DNA
tgaatcaaaccacccagctaaggggagg

SEQ ID NO: 30428 - DNA, 28 bp, synthetic construct
  source 1..28: mol_type = other DNA
gaatcaaaccacccagctaaggggaggg

SEQ ID NO: 30429 - DNA, 28 bp, synthetic construct
  source 1..28: mol_type = other DNA
accacccagctaaggggagggctgctgg

SEQ ID NO: 30430 - DNA, 28 bp, synthetic construct
  source 1..28: mol_type = other DNA
ccacccagctaaggggagggctgctggg

SEQ ID NO: 30431 - DNA, 28 bp, synthetic construct
  source 1..28: mol_type = other DNA
cacccagctaaggggagggctgctgggg

SEQ ID NO: 30432 - DNA, 28 bp, synthetic construct
  source 1..28: mol_type = other DNA
acccagctaaggggagggctgctggggg

SEQ ID NO: 30433 - DNA, 28 bp, synthetic construct
  source 1..28: mol_type = other DNA
tcccccagcagccctccccttagctggg

SEQ ID NO: 30434 - DNA, 28 bp, synthetic construct
  source 1..28: mol_type = other DNA
ttcccccagcagccctccccttagctgg

SEQ ID NO: 30435 - DNA, 28 bp, synthetic construct
  source 1..28: mol_type = other DNA
ctgctgggggaagctgctaaatgagagg

SEQ ID NO: 30436 - DNA, 28 bp, synthetic construct
  source 1..28: mol_type = other DNA
aagctgctaaatgagaggagctgcttgg

SEQ ID NO: 30437 - DNA, 28 bp, synthetic construct
  source 1..28: mol_type = other DNA
aaatgagaggagctgcttggcttcccgg

SEQ ID NO: 30438 - DNA, 28 bp, synthetic construct
  source 1..28: mol_type = other DNA
aatgagaggagctgcttggcttcccggg

SEQ ID NO: 30439 - DNA, 28 bp, synthetic construct
  source 1..28: mol_type = other DNA
gaggagctgcttggcttcccgggtcagg

SEQ ID NO: 30440 - DNA, 28 bp, synthetic construct
  source 1..28: mol_type = other DNA
agctgcttggcttcccgggtcaggttgg

SEQ ID NO: 30441 - DNA, 28 bp, synthetic construct
  source 1..28: mol_type = other DNA
gcttggcttcccgggtcaggttggttgg

SEQ ID NO: 30442 - DNA, 28 bp, synthetic construct
  source 1..28: mol_type = other DNA
ggcttcccgggtcaggttggttggttgg

SEQ ID NO: 30443 - DNA, 28 bp, synthetic construct
  source 1..28: mol_type = other DNA
ctacaccaaccaaccaacctgacccggg

SEQ ID NO: 30444 - DNA, 28 bp, synthetic construct
  source 1..28: mol_type = other DNA
tctacaccaaccaaccaacctgacccgg

SEQ ID NO: 30445 - DNA, 28 bp, synthetic construct
  source 1..28: mol_type = other DNA
ggtgtagactaaatgtaccaaagaaagg

SEQ ID NO: 30446 - DNA, 28 bp, synthetic construct
  source 1..28: mol_type = other DNA
gtgtagactaaatgtaccaaagaaaggg

SEQ ID NO: 30447 - DNA, 28 bp, synthetic construct
  source 1..28: mol_type = other DNA
ggattcatttgttagtccctttctttgg

SEQ ID NO: 30448 - DNA, 28 bp, synthetic construct
  source 1..28: mol_type = other DNA
actaacaaatgaatcctgctcagtctgg

SEQ ID NO: 30449 - DNA, 28 bp, synthetic construct
  source 1..28: mol_type = other DNA
ctaacaaatgaatcctgctcagtctggg

SEQ ID NO: 30450 - DNA, 28 bp, synthetic construct
  source 1..28: mol_type = other DNA
taacaaatgaatcctgctcagtctgggg

SEQ ID NO: 30451 - DNA, 28 bp, synthetic construct
  source 1..28: mol_type = other DNA
atgtgagtagggccccagactgagcagg

SEQ ID NO: 30452 - DNA, 28 bp, synthetic construct
  source 1..28: mol_type = other DNA
gcactaggttggcagaatgtgagtaggg

SEQ ID NO: 30453 - DNA, 28 bp, synthetic construct
  source 1..28: mol_type = other DNA
agcactaggttggcagaatgtgagtagg

SEQ ID NO: 30454 - DNA, 28 bp, synthetic construct
  source 1..28: mol_type = other DNA
tactcacattctgccaacctagtgctgg

SEQ ID NO: 30455 - DNA, 28 bp, synthetic construct
  source 1..28: mol_type = other DNA
atttaggaggcttccagcactaggttgg

SEQ ID NO: 30456 - DNA, 28 bp, synthetic construct
  source 1..28: mol_type = other DNA
atttatttaggaggcttccagcactagg

SEQ ID NO: 30457 - DNA, 28 bp, synthetic construct
  source 1..28: mol_type = other DNA
aggtttgcttctggatttatttaggagg

SEQ ID NO: 30458 - DNA, 28 bp, synthetic construct
  source 1..28: mol_type = other DNA
tataggtttgcttctggatttatttagg

SEQ ID NO: 30459 - DNA, 28 bp, synthetic construct
  source 1..28: mol_type = other DNA
atcttagatgctataggtttgcttctgg

SEQ ID NO: 30460 - DNA, 28 bp, synthetic construct
  source 1..28: mol_type = other DNA
tctgaagggagatcttagatgctatagg

SEQ ID NO: 30461 - DNA, 28 bp, synthetic construct
  source 1..28: mol_type = other DNA
tctcttctatcaaatcatatctgaaggg

SEQ ID NO: 30462 - DNA, 28 bp, synthetic construct
  source 1..28: mol_type = other DNA
ttctcttctatcaaatcatatctgaagg

SEQ ID NO: 30463 - DNA, 28 bp, synthetic construct
  source 1..28: mol_type = other DNA
gatttgatagaagagaagccttgcatgg

SEQ ID NO: 30464 - DNA, 28 bp, synthetic construct
  source 1..28: mol_type = other DNA
ataaggcatgaattaaagccatgcaagg

SEQ ID NO: 30465 - DNA, 28 bp, synthetic construct
  source 1..28: mol_type = other DNA
gagttgcagctgcgtcttcaggataagg

SEQ ID NO: 30466 - DNA, 28 bp, synthetic construct
  source 1..28: mol_type = other DNA
tcctgaagacgcagctgcaactcagagg

SEQ ID NO: 30467 - DNA, 28 bp, synthetic construct
  source 1..28: mol_type = other DNA
acctctgagttgcagctgcgtcttcagg

SEQ ID NO: 30468 - DNA, 28 bp, synthetic construct
  source 1..28: mol_type = other DNA
ctcagaggtcatttttgtaaccaagtgg

SEQ ID NO: 30469 - DNA, 28 bp, synthetic construct
  source 1..28: mol_type = other DNA
tcagaggtcatttttgtaaccaagtggg

SEQ ID NO: 30470 - DNA, 28 bp, synthetic construct
  source 1..28: mol_type = other DNA
ataaagagagaaaaaaaatcccacttgg

SEQ ID NO: 30471 - DNA, 28 bp, synthetic construct
  source 1..28: mol_type = other DNA
agacatatttttctaggggaatggtggg

SEQ ID NO: 30472 - DNA, 28 bp, synthetic construct
  source 1..28: mol_type = other DNA
cagacatatttttctaggggaatggtgg

SEQ ID NO: 30473 - DNA, 28 bp, synthetic construct
  source 1..28: mol_type = other DNA
caccattcccctagaaaaatatgtctgg

SEQ ID NO: 30474 - DNA, 28 bp, synthetic construct
  source 1..28: mol_type = other DNA
ggccagacatatttttctaggggaatgg

SEQ ID NO: 30475 - DNA, 28 bp, synthetic construct
  source 1..28: mol_type = other DNA
cttttggccagacatatttttctagggg

SEQ ID NO: 30476 - DNA, 28 bp, synthetic construct
  source 1..28: mol_type = other DNA
gcttttggccagacatatttttctaggg

SEQ ID NO: 30477 - DNA, 28 bp, synthetic construct
  source 1..28: mol_type = other DNA
agcttttggccagacatatttttctagg

SEQ ID NO: 30478 - DNA, 28 bp, synthetic construct
  source 1..28: mol_type = other DNA
tagaaaaatatgtctggccaaaagctgg

SEQ ID NO: 30479 - DNA, 28 bp, synthetic construct
  source 1..28: mol_type = other DNA
atgtctggccaaaagctggctctgcagg

SEQ ID NO: 30480 - DNA, 28 bp, synthetic construct
  source 1..28: mol_type = other DNA
tctggccaaaagctggctctgcaggtgg

SEQ ID NO: 30481 - DNA, 28 bp, synthetic construct
  source 1..28: mol_type = other DNA
cagtaccacctgcagagccagcttttgg

SEQ ID NO: 30482 - DNA, 28 bp, synthetic construct
  source 1..28: mol_type = other DNA
aagctggctctgcaggtggtactgctgg

SEQ ID NO: 30483 - DNA, 28 bp, synthetic construct
  source 1..28: mol_type = other DNA
tggctctgcaggtggtactgctggaagg

SEQ ID NO: 30484 - DNA, 28 bp, synthetic construct
  source 1..28: mol_type = other DNA
gcaggtggtactgctggaaggtgatagg

SEQ ID NO: 30485 - DNA, 28 bp, synthetic construct
  source 1..28: mol_type = other DNA
gctggaggagatgctgtaggggctgagg

SEQ ID NO: 30486 - DNA, 28 bp, synthetic construct
  source 1..28: mol_type = other DNA
gacaaagctggaggagatgctgtagggg

SEQ ID NO: 30487 - DNA, 28 bp, synthetic construct
  source 1..28: mol_type = other DNA
ggacaaagctggaggagatgctgtaggg

SEQ ID NO: 30488 - DNA, 28 bp, synthetic construct
  source 1..28: mol_type = other DNA
gggacaaagctggaggagatgctgtagg

SEQ ID NO: 30489 - DNA, 28 bp, synthetic construct
  source 1..28: mol_type = other DNA
agcatctcctccagctttgtccctaagg

SEQ ID NO: 30490 - DNA, 28 bp, synthetic construct
  source 1..28: mol_type = other DNA
gtagtgtccttagggacaaagctggagg

SEQ ID NO: 30491 - DNA, 28 bp, synthetic construct
  source 1..28: mol_type = other DNA
agagtagtgtccttagggacaaagctgg

SEQ ID NO: 30492 - DNA, 28 bp, synthetic construct
  source 1..28: mol_type = other DNA
ggaacaggagagagtagtgtccttaggg

SEQ ID NO: 30493 - DNA, 28 bp, synthetic construct
  source 1..28: mol_type = other DNA
tggaacaggagagagtagtgtccttagg

SEQ ID NO: 30494 - DNA, 28 bp, synthetic construct
  source 1..28: mol_type = other DNA
catgcgtctgcagctttgctggaacagg

SEQ ID NO: 30495 - DNA, 28 bp, synthetic construct
  source 1..28: mol_type = other DNA
tggagtcatgcgtctgcagctttgctgg

SEQ ID NO: 30496 - DNA, 28 bp, synthetic construct
  source 1..28: mol_type = other DNA
tgactccatctgcttctccttccagagg

SEQ ID NO: 30497 - DNA, 28 bp, synthetic construct
  source 1..28: mol_type = other DNA
agaagcctctggaaggagaagcagatgg

SEQ ID NO: 30498 - DNA, 28 bp, synthetic construct
  source 1..28: mol_type = other DNA
tctgcttctccttccagaggcttcttgg

SEQ ID NO: 30499 - DNA, 28 bp, synthetic construct
  source 1..28: mol_type = other DNA
ctgcttctccttccagaggcttcttggg

SEQ ID NO: 30500 - DNA, 28 bp, synthetic construct
  source 1..28: mol_type = other DNA
tacaaacacccaagaagcctctggaagg

SEQ ID NO: 30501 - DNA, 28 bp, synthetic construct
  source 1..28: mol_type = other DNA
cagttacaaacacccaagaagcctctgg

SEQ ID NO: 30502 - DNA, 28 bp, synthetic construct
  source 1..28: mol_type = other DNA
ttcttgggtgtttgtaactgtatccagg

SEQ ID NO: 30503 - DNA, 28 bp, synthetic construct
  source 1..28: mol_type = other DNA
tcttgggtgtttgtaactgtatccaggg

SEQ ID NO: 30504 - DNA, 28 bp, synthetic construct
  source 1..28: mol_type = other DNA
gtttgtaactgtatccagggattgcagg

SEQ ID NO: 30505 - DNA, 28 bp, synthetic construct
  source 1..28: mol_type = other DNA
ccagggattgcaggataaaccttctagg

SEQ ID NO: 30506 - DNA, 28 bp, synthetic construct
  source 1..28: mol_type = other DNA
gtaatttgcaaggagaaagcctagaagg

SEQ ID NO: 30507 - DNA, 28 bp, synthetic construct
  source 1..28: mol_type = other DNA
tcaacatattagcatgtaatttgcaagg

SEQ ID NO: 30508 - DNA, 28 bp, synthetic construct
  source 1..28: mol_type = other DNA
attacatgctaatatgttgaaccccagg

SEQ ID NO: 30509 - DNA, 28 bp, synthetic construct
  source 1..28: mol_type = other DNA
tggatctaaaatctacgctgtcctgggg

SEQ ID NO: 30510 - DNA, 28 bp, synthetic construct
  source 1..28: mol_type = other DNA
gtggatctaaaatctacgctgtcctggg

SEQ ID NO: 30511 - DNA, 28 bp, synthetic construct
  source 1..28: mol_type = other DNA
ggtggatctaaaatctacgctgtcctgg

SEQ ID NO: 30512 - DNA, 28 bp, synthetic construct
  source 1..28: mol_type = other DNA
gacagcgtagattttagatccacccagg

SEQ ID NO: 30513 - DNA, 28 bp, synthetic construct
  source 1..28: mol_type = other DNA
tccacccaggagttcttgtgtcttcagg

SEQ ID NO: 30514 - DNA, 28 bp, synthetic construct
  source 1..28: mol_type = other DNA
gcctgaagacacaagaactcctgggtgg

SEQ ID NO: 30515 - DNA, 28 bp, synthetic construct
  source 1..28: mol_type = other DNA
aaggcctgaagacacaagaactcctggg

SEQ ID NO: 30516 - DNA, 28 bp, synthetic construct
  source 1..28: mol_type = other DNA
aaaggcctgaagacacaagaactcctgg

SEQ ID NO: 30517 - DNA, 28 bp, synthetic construct
  source 1..28: mol_type = other DNA
ttcaggcctttccctctctctccacagg

SEQ ID NO: 30518 - DNA, 28 bp, synthetic construct
  source 1..28: mol_type = other DNA
gagatacctgtggagagagagggaaagg

SEQ ID NO: 30519 - DNA, 28 bp, synthetic construct
  source 1..28: mol_type = other DNA
actcagagatacctgtggagagagaggg

SEQ ID NO: 30520 - DNA, 28 bp, synthetic construct
  source 1..28: mol_type = other DNA
cactcagagatacctgtggagagagagg

SEQ ID NO: 30521 - DNA, 28 bp, synthetic construct
  source 1..28: mol_type = other DNA
ctctctctccacaggtatctctgagtgg

SEQ ID NO: 30522 - DNA, 28 bp, synthetic construct
  source 1..28: mol_type = other DNA
ggttagaaccactcagagatacctgtgg

SEQ ID NO: 30523 - DNA, 28 bp, synthetic construct
  source 1..28: mol_type = other DNA
aggtatctctgagtggttctaacctagg

SEQ ID NO: 30524 - DNA, 28 bp, synthetic construct
  source 1..28: mol_type = other DNA
ctgagtggttctaacctaggattcgagg

SEQ ID NO: 30525 - DNA, 28 bp, synthetic construct
  source 1..28: mol_type = other DNA
cagaaagaaaggcacctcgaatcctagg

SEQ ID NO: 30526 - DNA, 28 bp, synthetic construct
  source 1..28: mol_type = other DNA
gaatgatgaaaaaatacagaaagaaagg

SEQ ID NO: 30527 - DNA, 28 bp, synthetic construct
  source 1..28: mol_type = other DNA
tttctgtattttttcatcattcaccagg

SEQ ID NO: 30528 - DNA, 28 bp, synthetic construct
  source 1..28: mol_type = other DNA
catcattcaccaggtcccgagcagatgg

SEQ ID NO: 30529 - DNA, 28 bp, synthetic construct
  source 1..28: mol_type = other DNA
ttcaccaggtcccgagcagatggtgtgg

SEQ ID NO: 30530 - DNA, 28 bp, synthetic construct
  source 1..28: mol_type = other DNA
acagccacaccatctgctcgggacctgg

SEQ ID NO: 30531 - DNA, 28 bp, synthetic construct
  source 1..28: mol_type = other DNA
gtcagcacagccacaccatctgctcggg

SEQ ID NO: 30532 - DNA, 28 bp, synthetic construct
  source 1..28: mol_type = other DNA
agtcagcacagccacaccatctgctcgg

SEQ ID NO: 30533 - DNA, 28 bp, synthetic construct
  source 1..28: mol_type = other DNA
tgtcatcactcctcctatgtttccatgg

SEQ ID NO: 30534 - DNA, 28 bp, synthetic construct
  source 1..28: mol_type = other DNA
ctcctcctatgtttccatggaaacatgg

SEQ ID NO: 30535 - DNA, 28 bp, synthetic construct
  source 1..28: mol_type = other DNA
tcctcctatgtttccatggaaacatggg

SEQ ID NO: 30536 - DNA, 28 bp, synthetic construct
  source 1..28: mol_type = other DNA
ccccatgtttccatggaaacataggagg

SEQ ID NO: 30537 - DNA, 28 bp, synthetic construct
  source 1..28: mol_type = other DNA
atgccccatgtttccatggaaacatagg

SEQ ID NO: 30538 - DNA, 28 bp, synthetic construct
  source 1..28: mol_type = other DNA
atgtttccatggaaacatggggcatagg

SEQ ID NO: 30539 - DNA, 28 bp, synthetic construct
  source 1..28: mol_type = other DNA
tgtttccatggaaacatggggcataggg

SEQ ID NO: 30540 - DNA, 28 bp, synthetic construct
  source 1..28: mol_type = other DNA
atggtccctatgccccatgtttccatgg

SEQ ID NO: 30541 - DNA, 28 bp, synthetic construct
  source 1..28: mol_type = other DNA
tggggcatagggaccatctccgccttgg

SEQ ID NO: 30542 - DNA, 28 bp, synthetic construct
  source 1..28: mol_type = other DNA
ggggcatagggaccatctccgccttggg

SEQ ID NO: 30543 - DNA, 28 bp, synthetic construct
  source 1..28: mol_type = other DNA
actgtcagagagcccaaggcggagatgg

SEQ ID NO: 30544 - DNA, 28 bp, synthetic construct
  source 1..28: mol_type = other DNA
gaggatactgtcagagagcccaaggcgg

SEQ ID NO: 30545 - DNA, 28 bp, synthetic construct
  source 1..28: mol_type = other DNA
ccttgggctctctgacagtatcctctgg

SEQ ID NO: 30546 - DNA, 28 bp, synthetic construct
  source 1..28: mol_type = other DNA
cacaagtactgaagttcttcgccagagg

SEQ ID NO: 30547 - DNA, 28 bp, synthetic construct
  source 1..28: mol_type = other DNA
aggacagtggacaggctggggggagggg

SEQ ID NO: 30548 - DNA, 28 bp, synthetic construct
  source 1..28: mol_type = other DNA
taggacagtggacaggctggggggaggg

SEQ ID NO: 30549 - DNA, 28 bp, synthetic construct
  source 1..28: mol_type = other DNA
ctaggacagtggacaggctggggggagg

SEQ ID NO: 30550 - DNA, 28 bp, synthetic construct
  source 1..28: mol_type = other DNA
ctccccccagcctgtccactgtcctagg

SEQ ID NO: 30551 - DNA, 28 bp, synthetic construct
  source 1..28: mol_type = other DNA
tccccccagcctgtccactgtcctaggg

SEQ ID NO: 30552 - DNA, 28 bp, synthetic construct
  source 1..28: mol_type = other DNA
tccctaggacagtggacaggctgggggg

SEQ ID NO: 30553 - DNA, 28 bp, synthetic construct
  source 1..28: mol_type = other DNA
ctccctaggacagtggacaggctggggg

SEQ ID NO: 30554 - DNA, 28 bp, synthetic construct
  source 1..28: mol_type = other DNA
actccctaggacagtggacaggctgggg

SEQ ID NO: 30555 - DNA, 28 bp, synthetic construct
  source 1..28: mol_type = other DNA
aactccctaggacagtggacaggctggg

SEQ ID NO: 30556 - DNA, 28 bp, synthetic construct
  source 1..28: mol_type = other DNA
caactccctaggacagtggacaggctgg

SEQ ID NO: 30557 - DNA, 28 bp, synthetic construct
  source 1..28: mol_type = other DNA
cagcctgtccactgtcctagggagttgg

SEQ ID NO: 30558 - DNA, 28 bp, synthetic construct
  source 1..28: mol_type = other DNA
tctccaactccctaggacagtggacagg

SEQ ID NO: 30559 - DNA, 28 bp, synthetic construct
  source 1..28: mol_type = other DNA
aaaggtctccaactccctaggacagtgg

SEQ ID NO: 30560 - DNA, 28 bp, synthetic construct
  source 1..28: mol_type = other DNA
tgtcctagggagttggagacctttctgg

SEQ ID NO: 30561 - DNA, 28 bp, synthetic construct
  source 1..28: mol_type = other DNA
gtcctagggagttggagacctttctggg

SEQ ID NO: 30562 - DNA, 28 bp, synthetic construct
  source 1..28: mol_type = other DNA
tcctagggagttggagacctttctgggg

SEQ ID NO: 30563 - DNA, 28 bp, synthetic construct
  source 1..28: mol_type = other DNA
gccccagaaaggtctccaactccctagg

SEQ ID NO: 30564 - DNA, 28 bp, synthetic construct
  source 1..28: mol_type = other DNA
agacctttctggggccctagaagccagg

SEQ ID NO: 30565 - DNA, 28 bp, synthetic construct
  source 1..28: mol_type = other DNA
gacctttctggggccctagaagccaggg

SEQ ID NO: 30566 - DNA, 28 bp, synthetic construct
  source 1..28: mol_type = other DNA
gaccctggcttctagggccccagaaagg

SEQ ID NO: 30567 - DNA, 28 bp, synthetic construct
  source 1..28: mol_type = other DNA
atctctgaaatgaccctggcttctaggg

SEQ ID NO: 30568 - DNA, 28 bp, synthetic construct
  source 1..28: mol_type = other DNA
gatctctgaaatgaccctggcttctagg

SEQ ID NO: 30569 - DNA, 28 bp, synthetic construct
  source 1..28: mol_type = other DNA
ccttagatgatctctgaaatgaccctgg

SEQ ID NO: 30570 - DNA, 28 bp, synthetic construct
  source 1..28: mol_type = other DNA
catctaaggacatactccctgcaaatgg

SEQ ID NO: 30571 - DNA, 28 bp, synthetic construct
  source 1..28: mol_type = other DNA
atactccctgcaaatggttttgaactgg

SEQ ID NO: 30572 - DNA, 28 bp, synthetic construct
  source 1..28: mol_type = other DNA
tccctgcaaatggttttgaactggctgg

SEQ ID NO: 30573 - DNA, 28 bp, synthetic construct
  source 1..28: mol_type = other DNA
ccctgcaaatggttttgaactggctggg

SEQ ID NO: 30574 - DNA, 28 bp, synthetic construct
  source 1..28: mol_type = other DNA
tcccagccagttcaaaaccatttgcagg

SEQ ID NO: 30575 - DNA, 28 bp, synthetic construct
  source 1..28: mol_type = other DNA
aaatggttttgaactggctgggaaaagg

SEQ ID NO: 30576 - DNA, 28 bp, synthetic construct
  source 1..28: mol_type = other DNA
tggttttgaactggctgggaaaaggagg

SEQ ID NO: 30577 - DNA, 28 bp, synthetic construct
  source 1..28: mol_type = other DNA
ggttttgaactggctgggaaaaggaggg

SEQ ID NO: 30578 - DNA, 28 bp, synthetic construct
  source 1..28: mol_type = other DNA
tttgaactggctgggaaaaggagggagg

(The sequence listing continues in the following parts.)